European Patent Application EP 4 339 202 A1, published March 20, 2024. Title: FUSION PROTEINS COMPRISING GG REPEAT SEQUENCES II. Applicant: Numaferm GmbH. The sequence listing filed with the application follows.

SEQUENCE LISTING (50696 sequences)

SEQ ID NO: 1 - protein, 9 aa, synthetic construct
GGLGNDILT

SEQ ID NO: 2 - protein, 9 aa, synthetic construct
GGAGNDTLD

SEQ ID NO: 3 - protein, 9 aa, synthetic construct
GGAGNDTLN

SEQ ID NO: 4 - protein, 9 aa, synthetic construct
GGSGSDTYV

SEQ ID NO: 5 - protein, 9 aa, synthetic construct
GGAGNDYLE

SEQ ID NO: 6 - protein, 9 aa, synthetic construct
GGLGSDILT

SEQ ID NO: 7 - protein, 9 aa, synthetic construct
GGAGNDTLI

SEQ ID NO: 8 - protein, 9 aa, synthetic construct
GGSGNDKLS

SEQ ID NO: 9 - protein, 9 aa, synthetic construct
GGQGDDQLF

SEQ ID NO: 10 - protein, 9 aa, synthetic construct
GGEGNDYLN

SEQ ID NO: 11 - protein, 9 aa, synthetic construct
GGFGNDIYV

SEQ ID NO: 12 - protein, 9 aa, synthetic construct
GGGGIDLLD

SEQ ID NO: 13 - protein, 9 aa, synthetic construct
GGTGDDKLY

SEQ ID NO: 14 - protein, 9 aa, synthetic construct
GGEGDDVFK

SEQ ID NO: 15 - protein, 9 aa, synthetic construct
GGDGEDIFK

SEQ ID NO: 16 - protein, 9 aa, synthetic construct
GGAGNDTLT

SEQ ID NO: 17 - protein, 9 aa, synthetic construct
GGKGNDILL

SEQ ID NO: 18 - protein, 9 aa, synthetic construct
GGTGNDTLI

SEQ ID NO: 19 - protein, 9 aa, synthetic construct
GGAGNDTLV

SEQ ID NO: 20 - protein, 9 aa, synthetic construct
GGSGNDTLY

SEQ ID NO: 21 - protein, 9 aa, synthetic construct
GGDGNDLFY

SEQ ID NO: 22 - protein, 9 aa, synthetic construct
GGSGADTFV

SEQ ID NO: 23 - protein, 9 aa, synthetic construct
GGYGNDIYR

SEQ ID NO: 24 - protein, 9 aa, synthetic construct
GGGGVDTFF

SEQ ID NO: 25 - protein, 9 aa, synthetic construct
GGSGEDLFK

SEQ ID NO: 26 - protein, 9 aa, synthetic construct
GGQGNDTMT

SEQ ID NO: 27 - protein, 9 aa, synthetic construct
GGAGNDTLY

SEQ ID NO: 28 - protein, 9 aa, synthetic construct
GGNGDDQLY

SEQ ID NO: 29 - protein, 9 aa, synthetic construct
GGLGDDILT

SEQ ID NO: 30 - protein, 9 aa, synthetic construct
GGAGNDILY

SEQ ID NO: 31 - protein, 9 aa, synthetic construct
GGAGNDTLS

SEQ ID NO: 32 - protein, 9 aa, synthetic construct
GGDGNDKLI

SEQ ID NO: 33 - protein, 9 aa, synthetic construct
GGAGDDVLI

SEQ ID NO: 34 - protein, 9 aa, synthetic construct
GGEGNDLLK

SEQ ID NO: 35 - protein, 9 aa, synthetic construct
GGAGNDILV

SEQ ID NO: 36 - protein, 9 aa, synthetic construct
GGAGNDILI

SEQ ID NO: 37 - protein, 9 aa, synthetic construct
GGTGNDTLT

SEQ ID NO: 38 - protein, 9 aa, synthetic construct
GGAGADTLI

SEQ ID NO: 39 - protein, 9 aa, synthetic construct
GGGGADTFV

SEQ ID NO: 40 - protein, 9 aa, synthetic construct
GGAGNDVLI

SEQ ID NO: 41 - protein, 9 aa, synthetic construct
GGAGNDVLD

SEQ ID NO: 42 - protein, 9 aa, synthetic construct
GGTGNDTLD

SEQ ID NO: 43 - protein, 9 aa, synthetic construct
GGAGADTFV

SEQ ID NO: 44 - protein, 9 aa, synthetic construct
GGAGNDIIY

SEQ ID NO: 45 - protein, 9 aa, synthetic construct
GGAGADTLS

SEQ ID NO: 46 - protein, 9 aa, synthetic construct
GGAGNDTYI

SEQ ID NO: 47 - protein, 9 aa, synthetic construct
GGQGNDILI

SEQ ID NO: 48 - protein, 9 aa, synthetic construct
GGSGADTLI

SEQ ID NO: 49 - protein, 9 aa, synthetic construct
GGAGNDTYV

SEQ ID NO: 50 - protein, 9 aa, synthetic construct
GGEGNDGLR

SEQ ID NO: 51 - protein, 9 aa, synthetic construct
GGAGNDTLL

SEQ ID NO: 52 - protein, 9 aa, synthetic construct
GGLGNDILV

SEQ ID NO: 53 - protein, 9 aa, synthetic construct
GGAGADKLT

SEQ ID NO: 54 - protein, 9 aa, synthetic construct
GGAGDDLLI

SEQ ID NO: 55 - protein, 9 aa, synthetic construct
GGAGADTLD

SEQ ID NO: 56 - protein, 9 aa, synthetic construct
GGAGDDTLD

SEQ ID NO: 57 - protein, 9 aa, synthetic construct
GGAGNDLLD

SEQ ID NO: 58 - protein, 9 aa, synthetic construct
GGAGDDILV

SEQ ID NO: 59 - protein, 9 aa, synthetic construct
GGKGNDTIR

SEQ ID NO: 60 - protein, 9 aa, synthetic construct
GGAGDDTLV

SEQ ID NO: 61 - protein, 9 aa, synthetic construct
GGAGNDILF

SEQ ID NO: 62 - protein, 9 aa, synthetic construct
GGSGNDTLL

SEQ ID NO: 63 - protein, 9 aa, synthetic construct
GGAGNDVLF

SEQ ID NO: 64 - protein, 9 aa, synthetic construct
GGAGNDRLD

SEQ ID NO: 65 - protein, 9 aa, synthetic construct
GGDGNDTLS

SEQ ID NO: 66 - protein, 9 aa, synthetic construct
GGAGNDILN

SEQ ID NO: 67 - protein, 9 aa, synthetic construct
GGDGNDLLI

SEQ ID NO: 68 - protein, 9 aa, synthetic construct
GGAGDDTLT

SEQ ID NO: 69 - protein, 9 aa, synthetic construct
GGAGDDTYI

SEQ ID NO: 70 - protein, 9 aa, synthetic construct
GGSGDDVII

SEQ ID NO: 71 - protein, 9 aa, synthetic construct
GGSGNDQLY

SEQ ID NO: 72 - protein, 9 aa, synthetic construct
GGLGNDYLD

SEQ ID NO: 73 - protein, 9 aa, synthetic construct
GGAGNDVLN

SEQ ID NO: 74 - protein, 9 aa, synthetic construct
GGGGDDLLI

SEQ ID NO: 75 - protein, 9 aa, synthetic construct
GGSGNDTLI

SEQ ID NO: 76 - protein, 9 aa, synthetic construct
GGNGDDILA

SEQ ID NO: 77 - protein, 9 aa, synthetic construct
GGLGADQLW

SEQ ID NO: 78 - protein, 9 aa, synthetic construct
GGDGNDALR

SEQ ID NO: 79 - protein, 9 aa, synthetic construct
GGLGNDTLN

SEQ ID NO: 80 - protein, 9 aa, synthetic construct
GGLGADSMT

SEQ ID NO: 81 - protein, 9 aa, synthetic construct
GGAGADTLT

SEQ ID NO: 82 - protein, 9 aa, synthetic construct
GGAGNDSLS

SEQ ID NO: 83 - protein, 9 aa, synthetic construct
GGAGNDVLT

SEQ ID NO: 84 - protein, 9 aa, synthetic construct
GGDGDDILI

SEQ ID NO: 85 - protein, 9 aa, synthetic construct
GGAGADVLD

SEQ ID NO: 86 - protein, 9 aa, synthetic construct
GGLGNDTYR

SEQ ID NO: 87 - protein, 9 aa, synthetic construct
GGAGNDILD

SEQ ID NO: 88 - protein, 9 aa, synthetic construct
GGDGNDTLI

SEQ ID NO: 89 - protein, 9 aa, synthetic construct
GGGGADQLW

SEQ ID NO: 90 - protein, 9 aa, synthetic construct
GGIGNDFLD

SEQ ID NO: 91 - protein, 9 aa, synthetic construct
GGLGNDILI

SEQ ID NO: 92 - protein, 9 aa, synthetic construct
GGDGNDTLL

SEQ ID NO: 93 - protein, 9 aa, synthetic construct
GGDGADIFK

SEQ ID NO: 94 - protein, 9 aa, synthetic construct
GGTGADTFV

SEQ ID NO: 95 - protein, 9 aa, synthetic construct
GGAGSDTFK

SEQ ID NO: 96 - protein, 9 aa, synthetic construct
GGLGNDTLI

SEQ ID NO: 97 - protein, 9 aa, synthetic construct
GGAGNDTLF

SEQ ID NO: 98 - protein, 9 aa, synthetic construct
GGNGNDILI

SEQ ID NO: 99 - protein, 9 aa, synthetic construct
GGDGNDLLR

SEQ ID NO: 100 - protein, 9 aa, synthetic construct
GGGGNDTLI

SEQ ID NO: 101 - protein, 9 aa, synthetic construct
GGLGDDYLD

SEQ ID NO: 102 - protein, 9 aa, synthetic construct
GGAGNDLME

SEQ ID NO: 103 - protein, 9 aa, synthetic construct
GGDGNDRLF

SEQ ID NO: 104 - protein, 9 aa, synthetic construct
GGAGNDTID

SEQ ID NO: 105 - protein, 9 aa, synthetic construct
GGLGADTLI

SEQ ID NO: 106 - protein, 9 aa, synthetic construct
GGAGNDLLY

SEQ ID NO: 107 - protein, 9 aa, synthetic construct
GGSGNDTLD

SEQ ID NO: 108 - protein, 9 aa, synthetic construct
GGSGNDILI

SEQ ID NO: 109 - protein, 9 aa, synthetic construct
GGDGNDTLD

SEQ ID NO: 110 - protein, 9 aa, synthetic construct
GGAGNDTFV

SEQ ID NO: 111 - protein, 9 aa, synthetic construct
GGAGNDLLI

SEQ ID NO: 112 - protein, 9 aa, synthetic construct
GGKGADFIE

SEQ ID NO: 113 - protein, 9 aa, synthetic construct
GGAGDDLLD

SEQ ID NO: 114 - protein, 9 aa, synthetic construct
GGAGQDTLI

SEQ ID NO: 115 - protein, 9 aa, synthetic construct
GGAGDDVLY

SEQ ID NO: 116 - protein, 9 aa, synthetic construct
GGSGNDTLS

SEQ ID NO: 117 - protein, 9 aa, synthetic construct
GGAGADTFR

SEQ ID NO: 118 - protein, 9 aa, synthetic construct
GGVGNDVMI

SEQ ID NO: 119 - protein, 9 aa, synthetic construct
GGDGADNLQ

SEQ ID NO: 120 - protein, 9 aa, synthetic construct
GGSGDDRLI

SEQ ID NO: 121 - protein, 9 aa, synthetic construct
GGAGRDSLY

SEQ ID NO: 122 - protein, 9 aa, synthetic construct
GGDGADTFR

SEQ ID NO: 123 - protein, 9 aa, synthetic construct
GGGGADTFI

SEQ ID NO: 124 - protein, 9 aa, synthetic construct
GGTGSDTLT

SEQ ID NO: 125 - protein, 9 aa, synthetic construct
GGAGNDVFV

SEQ ID NO: 126 - protein, 9 aa, synthetic construct
GGAGDDKLD

SEQ ID NO: 127 - protein, 9 aa, synthetic construct
GGAGADRLD

SEQ ID NO: 128 - protein, 9 aa, synthetic construct
GGAGNDVIY

SEQ ID NO: 129 - protein, 9 aa, synthetic construct
GGAGNDTLE

SEQ ID NO: 130 - protein, 9 aa, synthetic construct
GGAGNDTLA

SEQ ID NO: 131 - protein, 9 aa, synthetic construct
GGDGNDTLN

SEQ ID NO: 132 - protein, 9 aa, synthetic construct
GGTGNDTLN

SEQ ID NO: 133 - protein, 9 aa, synthetic construct
GGAGNDTIN

SEQ ID NO: 134 - protein, 9 aa, synthetic construct
GGAGADSLI

SEQ ID NO: 135 - protein, 9 aa, synthetic construct
GGLGNDILK

SEQ ID NO: 136 - protein, 9 aa, synthetic construct
GGTGNDTYV

SEQ ID NO: 137 - protein, 9 aa, synthetic construct
GGAGDDTLI

SEQ ID NO: 138 - protein, 9 aa, synthetic construct
GGLGHDILT

SEQ ID NO: 139 - protein, 9 aa, synthetic construct
GGSGDDILI

SEQ ID NO: 140 - protein, 9 aa, synthetic construct
GGLGNDTLT

SEQ ID NO: 141 - protein, 9 aa, synthetic construct
GGAGDDVLD

SEQ ID NO: 142 - protein, 9 aa, synthetic construct
GGAGNDLIY

SEQ ID NO: 143 - protein, 9 aa, synthetic construct
GGGGNDYLY

SEQ ID NO: 144 - protein, 9 aa, synthetic construct
GGAGNDSLY

SEQ ID NO: 145 - protein, 9 aa, synthetic construct
GGAGNDTIT

SEQ ID NO: 146 - protein, 9 aa, synthetic construct
GGLGNDHLY

SEQ ID NO: 147 - protein, 9 aa, synthetic construct
GGAGSDLLI

SEQ ID NO: 148 - protein, 9 aa, synthetic construct
GGAGNDTYY

SEQ ID NO: 149 - protein, 9 aa, synthetic construct
GGEGDDVLL

SEQ ID NO: 150 - protein, 9 aa, synthetic construct
GGEGNDTLI

SEQ ID NO: 151 - protein, 9 aa, synthetic construct
GGDGNDILI

SEQ ID NO: 152 - protein, 9 aa, synthetic construct
GGAGDDILI

SEQ ID NO: 153 - protein, 9 aa, synthetic construct
GGDGNDTLY

SEQ ID NO: 154 - protein, 9 aa, synthetic construct
GGAGQDYLD

SEQ ID NO: 155 - protein, 9 aa, synthetic construct
GGDGDDLLF

SEQ ID NO: 156 - protein, 9 aa, synthetic construct
GGDGDDRLF

SEQ ID NO: 157 - protein, 9 aa, synthetic construct
GGAGNDKLV

SEQ ID NO: 158 - protein, 9 aa, synthetic construct
GGTGADHYV

SEQ ID NO: 159 - protein, 9 aa, synthetic construct
GGDGNDTIN

SEQ ID NO: 160 - protein, 9 aa, synthetic construct
GGAGADTFK

SEQ ID NO: 161 - protein, 9 aa, synthetic construct
GGAGNDLLE

SEQ ID NO: 162 - protein, 9 aa, synthetic construct
GGDGNDVLR

SEQ ID NO: 163 - protein, 9 aa, synthetic construct
GGAGMDTLT

SEQ ID NO: 164 - protein, 9 aa, synthetic construct
GGQGNDTYI

SEQ ID NO: 165 - protein, 9 aa, synthetic construct
GGQGNDILD

SEQ ID NO: 166 - protein, 9 aa, synthetic construct
GGAGNDVIV

SEQ ID NO: 167 - protein, 9 aa, synthetic construct
GGAGNDLIL

SEQ ID NO: 168 - protein, 9 aa, synthetic construct
GGTGNDTLS

SEQ ID NO: 169 - protein, 9 aa, synthetic construct
GGAGNDTLR

SEQ ID NO: 170 - protein, 9 aa, synthetic construct
GGAGNDRLE

SEQ ID NO: 171 - protein, 9 aa, synthetic construct
GGAGADKLS

SEQ ID NO: 172 - protein, 9 aa, synthetic construct
GGLGSDTMT

SEQ ID NO: 173 - protein, 9 aa, synthetic construct
GGGGADELW

SEQ ID NO: 174 - protein, 9 aa, synthetic construct
GGAGDDTLN

SEQ ID NO: 175 - protein, 9 aa, synthetic construct
GGNGNDALY

SEQ ID NO: 176 - protein, 9 aa, synthetic construct
GGDGNDMLY

SEQ ID NO: 177 - protein, 9 aa, synthetic construct
GGAGNDTAD

SEQ ID NO: 178 - protein, 9 aa, synthetic construct
GGLGNDTYI

SEQ ID NO: 179 - protein, 9 aa, synthetic construct
GGAGNDYLD

SEQ ID NO: 180 - protein, 9 aa, synthetic construct
GGTGADTFR

SEQ ID NO: 181 - protein, 9 aa, synthetic construct
GGKGNDTLI

SEQ ID NO: 182 - protein, 9 aa, synthetic construct
GGLGDDTLE

SEQ ID NO: 183 - protein, 9 aa, synthetic construct
GGAGADTLR

SEQ ID NO: 184 - protein, 9 aa, synthetic construct
GGLGADVLD

SEQ ID NO: 185 - protein, 9 aa, synthetic construct
GGIGDDILH

SEQ ID NO: 186 - protein, 9 aa, synthetic construct
GGSGNDTLN

SEQ ID NO: 187 - protein, 9 aa, synthetic construct
GGAGNDRMW

SEQ ID NO: 188 - protein, 9 aa, synthetic construct
GGAGDDRLD

SEQ ID NO: 189 - protein, 9 aa, synthetic construct
GGEGNDTLL

SEQ ID NO: 190 - protein, 9 aa, synthetic construct
GGLGNDTYV

SEQ ID NO: 191 - protein, 9 aa, synthetic construct
GGAGNDWFG

SEQ ID NO: 192 - protein, 9 aa, synthetic construct
GGAGADTLV

SEQ ID NO: 193 - protein, 9 aa, synthetic construct
GGAGNDILT

SEQ ID NO: 194 - protein, 9 aa, synthetic construct
GGAGADTLN

SEQ ID NO: 195 - protein, 9 aa, synthetic construct
GGAGADKLD

SEQ ID NO: 196 - protein, 9 aa, synthetic construct
GGTGNDTYI

SEQ ID NO: 197 - protein, 9 aa, synthetic construct
GGMGNDILH

SEQ ID NO: 198 - protein, 9 aa, synthetic construct
GGGGADRLN

SEQ ID NO: 199 - protein, 9 aa, synthetic construct
GGAGNDRLI

SEQ ID NO: 200 - protein, 9 aa, synthetic construct
GGAGNDVLV

SEQ ID NO: 201 - protein, 9 aa, synthetic construct
GGAGNDSLD

SEQ ID NO: 202 - protein, 9 aa, synthetic construct
GGSGDDILV

SEQ ID NO: 203 - protein, 9 aa, synthetic construct
GGAGNDNLS

SEQ ID NO: 204 - protein, 9 aa, synthetic construct
GGTGADRYV

SEQ ID NO: 205 - protein, 9 aa, synthetic construct
GGDGDDTLI

SEQ ID NO: 206 - protein, 9 aa, synthetic construct
GGLGNDYMD

SEQ ID NO: 207 - protein, 9 aa, synthetic construct
GGTGVDKLT

SEQ ID NO: 208 - protein, 9 aa, synthetic construct
GGSGNDTLT

SEQ ID NO: 209 - protein, 9 aa, synthetic construct
GGSGDDTLS

SEQ ID NO: 210 - protein, 9 aa, synthetic construct
GGGGNDVLD

SEQ ID NO: 211 - protein, 9 aa, synthetic construct
GGEGNDTLD

SEQ ID NO: 212 - protein, 9 aa, synthetic construct
GGAGDDLLV

SEQ ID NO: 213 - protein, 9 aa, synthetic construct
GGNGNDTLD

SEQ ID NO: 214 - protein, 9 aa, synthetic construct
GGAGNDTYL

SEQ ID NO: 215 - protein, 9 aa, synthetic construct
GGSGNDTLF

SEQ ID NO: 216 - protein, 9 aa, synthetic construct
GGAGADRFV

SEQ ID NO: 217 - protein, 9 aa, synthetic construct
GGGGNDTLD

SEQ ID NO: 218 - protein, 9 aa, synthetic construct
GGSGDDRLD

SEQ ID NO: 219 - protein, 9 aa, synthetic construct
GGGGADKLW

SEQ ID NO: 220 - protein, 9 aa, synthetic construct
GGTGNDTLY

SEQ ID NO: 221 - protein, 9 aa, synthetic construct
GGAGADTLL

SEQ ID NO: 222 - protein, 9 aa, synthetic construct
GGTGNDTLF

SEQ ID NO: 223 - protein, 9 aa, synthetic construct
GGAGTDNLT

SEQ ID NO: 224 - protein, 9 aa, synthetic construct
GGAGDDTYV

SEQ ID NO: 225 - protein, 9 aa, synthetic construct
GGSGNDHLY

SEQ ID NO: 226 - protein, 9 aa, synthetic construct
GGDGDDVLD

SEQ ID NO: 227 - protein, 9 aa, synthetic construct
GGKGDDTLI

SEQ ID NO: 228 - protein, 9 aa, synthetic construct
GGAGDDVLV

SEQ ID NO: 229 - protein, 9 aa, synthetic construct
GGEGIDTFT

SEQ ID NO: 230 - protein, 9 aa, synthetic construct
GGLGNDKLI

SEQ ID NO: 231 - protein, 9 aa, synthetic construct
GGAGNDVLL

SEQ ID NO: 232 - protein, 9 aa, synthetic construct
GGGGADSLT

SEQ ID NO: 233 - protein, 9 aa, synthetic construct
GGNGNDTLE

SEQ ID NO: 234 - protein, 9 aa, synthetic construct
GGSGADILR

SEQ ID NO: 235 - protein, 9 aa, synthetic construct
GGAGADVFR

SEQ ID NO: 236 - protein, 9 aa, synthetic construct
GGTGADTYA

SEQ ID NO: 237 - protein, 9 aa, synthetic construct
GGDGDDQLS

SEQ ID NO: 238 - protein, 9 aa, synthetic construct
GGAGNDILR

SEQ ID NO: 239 - protein, 9 aa, synthetic construct
GGGGADTLT

SEQ ID NO: 240 - protein, 9 aa, synthetic construct
GGAGNDVLY

SEQ ID NO: 241 - protein, 9 aa, synthetic construct
GGNGNDILN

SEQ ID NO: 242 - protein, 9 aa, synthetic construct
GGGGNDTIL

SEQ ID NO: 243 - protein, 9 aa, synthetic construct
GGAGADLLD

SEQ ID NO: 244 - protein, 9 aa, synthetic construct
GGAGIDKLT

SEQ ID NO: 245 - protein, 9 aa, synthetic construct
GGKGADQLW

SEQ ID NO: 246 - protein, 9 aa, synthetic construct
GGAGNDRLY

SEQ ID NO: 247 - protein, 9 aa, synthetic construct
GGAGADVFV

SEQ ID NO: 248 - protein, 9 aa, synthetic construct
GGAGDDILN

SEQ ID NO: 249 - protein, 9 aa, synthetic construct
GGDGADTFV

SEQ ID NO: 250 - protein, 9 aa, synthetic construct
GGAGADQFI

SEQ ID NO: 251 - protein, 9 aa, synthetic construct
GGEGNDLLI

SEQ ID NO: 252 - protein, 9 aa, synthetic construct
GGAGNDLLH

SEQ ID NO: 253 - protein, 9 aa, synthetic construct
GGVGSDLFV

SEQ ID NO: 254 - protein, 9 aa, synthetic construct
GGDGDDILV

SEQ ID NO: 255 - protein, 9 aa, synthetic construct
GGGGADTLI

SEQ ID NO: 256 - protein, 9 aa, synthetic construct
GGAGNDVLS

SEQ ID NO: 257 - protein, 9 aa, synthetic construct
GGAGNDYLN

SEQ ID NO: 258 - protein, 9 aa, synthetic construct
GGDGNDTLT

SEQ ID NO: 259 - protein, 9 aa, synthetic construct
GGAGADTLA

SEQ ID NO: 260 - protein, 9 aa, synthetic construct
GGEGDDRLF

SEQ ID NO: 261 - protein, 9 aa, synthetic construct
GGSGDDDLY

SEQ ID NO: 262 - protein, 9 aa, synthetic construct
GGSGDDYLD

SEQ ID NO: 263 - protein, 9 aa, synthetic construct
GGDGDDTLL

SEQ ID NO: 264 - protein, 9 aa, synthetic construct
GGAGNDLLS

SEQ ID NO: 265 - protein, 9 aa, synthetic construct
GGTGNDTLL

SEQ ID NO: 266 - protein, 9 aa, synthetic construct
GGKGNDTLT

SEQ ID NO: 267 - protein, 9 aa, synthetic construct
GGAGNDTIL

SEQ ID NO: 268 - protein, 9 aa, synthetic construct
GGLGNDTLS

SEQ ID NO: 269 - protein, 9 aa, synthetic construct
GGAGQDQLW

SEQ ID NO: 270 - protein, 9 aa, synthetic construct
GGTGNDRFV

SEQ ID NO: 271 - protein, 9 aa, synthetic construct
GGAGDDTIF

SEQ ID NO: 272 - protein, 9 aa, synthetic construct
GGDGHDRLY

SEQ ID NO: 273 - protein, 9 aa, synthetic construct
GGGGNDTLL

SEQ ID NO: 274 - protein, 9 aa, synthetic construct
GGAGDDVLS

SEQ ID NO: 275 - protein, 9 aa, synthetic construct
GGAGDDTLS

SEQ ID NO: 276 - protein, 9 aa, synthetic construct
GGAGGDTLI

SEQ ID NO: 277 - protein, 9 aa, synthetic construct
GGAGADTLY

SEQ ID NO: 278 - protein, 9 aa, synthetic construct
GGTGTDSFD

SEQ ID NO: 279 - protein, 9 aa, synthetic construct
GGDGSDSYY

SEQ ID NO: 280 - protein, 9 aa, synthetic construct
GGTGNDTAS

SEQ ID NO: 281 - protein, 9 aa, synthetic construct
GGAGADTMI

SEQ ID NO: 282 - protein, 9 aa, synthetic construct
GGLGDDYLL

SEQ ID NO: 283 - protein, 9 aa, synthetic construct
GGAGNDLLV

SEQ ID NO: 284 - protein, 9 aa, synthetic construct
GGDGDDTLY

SEQ ID NO: 285 - protein, 9 aa, synthetic construct
GGAGNDTII

SEQ ID NO: 286 - protein, 9 aa, synthetic construct
GGAGDDILD

SEQ ID NO: 287 - protein, 9 aa, synthetic construct
GGLGNDTLD

SEQ ID NO: 288 - protein, 9 aa, synthetic construct
GGNGNDLLI

SEQ ID NO: 289 - protein, 9 aa, synthetic construct
GGIGNDILQ

SEQ ID NO: 290 - protein, 9 aa, synthetic construct
GGAGDDILT

SEQ ID NO: 291 - protein, 9 aa, synthetic construct
GGAGADRLI

SEQ ID NO: 292 - protein, 9 aa, synthetic construct
GGAGNDTIY

SEQ ID NO: 293 - protein, 9 aa, synthetic construct
GGKGNDVLV

SEQ ID NO: 294 - protein, 9 aa, synthetic construct
GGDGNDVLD

SEQ ID NO: 295 - protein, 9 aa, synthetic construct
GGAGADHME

SEQ ID NO: 296 - protein, 9 aa, synthetic construct
GGDGNDTLV

SEQ ID NO: 297 - protein, 9 aa, synthetic construct
GGGGNDTLN

SEQ ID NO: 298 - protein, 9 aa, synthetic construct
GGSGADQFV

SEQ ID NO: 299 - protein, 9 aa, synthetic construct
GGAGDDRII

SEQ ID NO: 300 - protein, 9 aa, synthetic construct
GGSGNDTLV

SEQ ID NO: 301 - protein, 9 aa, synthetic construct
GGTGFDYLV

SEQ ID NO: 302 - protein, 9 aa, synthetic construct
GGNGNDTAS

SEQ ID NO: 303 - protein, 9 aa, synthetic construct
GGLGNDVLN

SEQ ID NO: 304 - protein, 9 aa, synthetic construct
GGAGNDVLR

SEQ ID NO: 305 - protein, 9 aa, synthetic construct
GGTGHDVFV

SEQ ID NO: 306 - protein, 9 aa, synthetic construct
GGAGNDRLF

SEQ ID NO: 307 - protein, 9 aa, synthetic construct
GGAGDDRLF

SEQ ID NO: 308 - protein, 9 aa, synthetic construct
GGVGNDTLD

SEQ ID NO: 309 - protein, 9 aa, synthetic construct
GGAGDDKLY

SEQ ID NO: 310 - protein, 9 aa, synthetic construct
GGAGNDRLS

SEQ ID NO: 311 - protein, 9 aa, synthetic construct
GGLGNDVLY

SEQ ID NO: 312 - protein, 9 aa, synthetic construct
GGAGDDTLL

SEQ ID NO: 313 - protein, 9 aa, synthetic construct
GGGGNDKIE

SEQ ID NO: 314 - protein, 9 aa, synthetic construct
GGAGADSFV

SEQ ID NO: 315 - protein, 9 aa, synthetic construct
GGEGDDLLI

SEQ ID NO: 316 - protein, 9 aa, synthetic construct
GGSGNDTLE

SEQ ID NO: 317 - protein, 9 aa, synthetic construct
GGLGDDILI

SEQ ID NO: 318 - protein, 9 aa, synthetic construct
GGAGNDSLT

SEQ ID NO: 319 - protein, 9 aa, synthetic construct
GGAGNDFLF

SEQ ID NO: 320 - protein, 9 aa, synthetic construct
GGVGNDTLN

SEQ ID NO: 321 - protein, 9 aa, synthetic construct
GGYGNDELR

SEQ ID NO: 322 - protein, 9 aa, synthetic construct
GGGGNDIFK

SEQ ID NO: 323 - protein, 9 aa, synthetic construct
GGEGDDVLI

SEQ ID NO: 324 - protein, 9 aa, synthetic construct
GGNGNDVLI

SEQ ID NO: 325 - protein, 9 aa, synthetic construct
GGAGDDTLY

SEQ ID NO: 326 - protein, 9 aa, synthetic construct
GGAGNDALD

SEQ ID NO: 327 - protein, 9 aa, synthetic construct
GGAGADSLD

SEQ ID NO: 328 - protein, 9 aa, synthetic construct
GGSGDDTLI

SEQ ID NO: 329 - protein, 9 aa, synthetic construct
GGAGNDLLN

SEQ ID NO: 330 - protein, 9 aa, synthetic construct
GGGGGDTLW

SEQ ID NO: 331 - protein, 9 aa, synthetic construct
GGAGNDTLQ

SEQ ID NO: 332 - protein, 9 aa, synthetic construct
GGLGQDTLT

SEQ ID NO: 333 - protein, 9 aa, synthetic construct
GGTGNDTYF

SEQ ID NO: 334 - protein, 9 aa, synthetic construct
GGAGNDKLY

SEQ ID NO: 335 - protein, 9 aa, synthetic construct
GGLGNDYLY

SEQ ID NO: 336 - protein, 9 aa, synthetic construct
GGDGNDYLD

SEQ ID NO: 337 - protein, 9 aa, synthetic construct
GGAGDDILY

SEQ ID NO: 338 - protein, 9 aa, synthetic construct
GGLGADIMT

SEQ ID NO: 339 - protein, 9 aa, synthetic construct
GGDGVDNLQ

SEQ ID NO: 340 - protein, 9 aa, synthetic construct
GGAGNDVIW

SEQ ID NO: 341 - protein, 9 aa, synthetic construct
GGLGGDTFV

SEQ ID NO: 342 - protein, 9 aa, synthetic construct
GGDGNDEIY

SEQ ID NO: 343 - protein, 9 aa, synthetic construct
GGNGNDTLI

SEQ ID NO: 344 - protein, 9 aa, synthetic construct
GGAGDDVIY

SEQ ID NO: 345 - protein, 9 aa, synthetic construct
GGKGNDILT

SEQ ID NO: 346 - protein, 9 aa, synthetic construct
GGAGNDVLM

SEQ ID NO: 347 - protein, 9 aa, synthetic construct
GGAGNDILS

SEQ ID NO: 348 - protein, 9 aa, synthetic construct
GGDGADFVN

SEQ ID NO: 349 - protein, 9 aa, synthetic construct
GGDGNDRLV

SEQ ID NO: 350 - protein, 9 aa, synthetic construct
GGKGADSLI

SEQ ID NO: 351 - protein, 9 aa, synthetic construct
GGTGNDILT

SEQ ID NO: 352 - protein, 9 aa, synthetic construct
GGDGDDVLI

SEQ ID NO: 353 - protein, 9 aa, synthetic construct
GGAGADLME

SEQ ID NO: 354 - protein, 9 aa, synthetic construct
GGYGDDTYL

SEQ ID NO: 355 - protein, 9 aa, synthetic construct
GGAGDDTID

SEQ ID NO: 356 - protein, 9 aa, synthetic construct
GGHGDDTVF

SEQ ID NO: 357 - protein, 9 aa, synthetic construct
GGAGNDTLH

SEQ ID NO: 358 - protein, 9 aa, synthetic construct
GGAGIDTAV

SEQ ID NO: 359 - protein, 9 aa, synthetic construct
GGKGNDVFV

SEQ ID NO: 360 - protein, 9 aa, synthetic construct
GGAGADRLT

SEQ ID NO: 361 - protein, 9 aa, synthetic construct
GGDGNDVLI

SEQ ID NO: 362 - protein, 9 aa, synthetic construct
GGDGDDTLD

SEQ ID NO: 363 - protein, 9 aa, synthetic construct
GGSGNDTIT

SEQ ID NO: 364 - protein, 9 aa, synthetic construct
GGAGNDLLR

SEQ ID NO: 365 - protein, 9 aa, synthetic construct
GGKGGDYIE

SEQ ID NO: 366 - protein, 9 aa, synthetic construct
GGAGNDSLN

SEQ ID NO: 367 - protein, 9 aa, synthetic construct
GGTGNDILS

SEQ ID NO: 368 - protein, 9 aa, synthetic construct
GGTGADTFK

SEQ ID NO: 369 - protein, 9 aa, synthetic construct
GGGGNDMMF

SEQ ID NO: 370 - protein, 9 aa, synthetic construct
GGSGDDELN

SEQ ID NO: 371 - protein, 9 aa, synthetic construct
GGGGADTLD

SEQ ID NO: 372 - protein, 9 aa, synthetic construct
GGQGDDILI

SEQ ID NO: 373 - protein, 9 aa, synthetic construct
GGDGDDTLS

SEQ ID NO: 374 - protein, 9 aa, synthetic construct
GGSGNDVLD

SEQ ID NO: 375 - protein, 9 aa, synthetic construct
GGLGDDIYY

SEQ ID NO: 376 - protein, 9 aa, synthetic construct
GGSGIDTVV

SEQ ID NO: 377 - protein, 9 aa, synthetic construct
GGAGGDLLK

SEQ ID NO: 378 - protein, 9 aa, synthetic construct
GGDGDDLLD

SEQ ID NO: 379 - protein, 9 aa, synthetic construct
GGAGDDVLT

SEQ ID NO: 380 - protein, 9 aa, synthetic construct
GGAGIDTLI

SEQ ID NO: 381 - protein, 9 aa, synthetic construct
GGDGNDRLY

SEQ ID NO: 382 - protein, 9 aa, synthetic construct
GGNGDDTLN

SEQ ID NO: 383 - protein, 9 aa, synthetic construct
GGAGDDVLA

SEQ ID NO: 384 - protein, 9 aa, synthetic construct
GGQGNDTLI

SEQ ID NO: 385 - protein, 9 aa, synthetic construct
GGTGNDSLI

SEQ ID NO: 386 - protein, 9 aa, synthetic construct
GGAGADLLI

SEQ ID NO: 387 - protein, 9 aa, synthetic construct
GGNGNDTLY

SEQ ID NO: 388 - protein, 9 aa, synthetic construct
GGPGDDVLT

SEQ ID NO: 389 - protein, 9 aa, synthetic construct
GGAGNDKLT

SEQ ID NO: 390 - protein, 9 aa, synthetic construct
GGLGADILV

SEQ ID NO: 391 - protein, 9 aa, synthetic construct
GGDGNDTID

SEQ ID NO: 392 - protein, 9 aa, synthetic construct
GGKGNDTLR

SEQ ID NO: 393 - protein, 9 aa, synthetic construct
GGTGDDTLY

SEQ ID NO: 394 - protein, 9 aa, synthetic construct
GGAGADIFQ

SEQ ID NO: 395 - protein, 9 aa, synthetic construct
GGSGNDKLY

SEQ ID NO: 396 - protein, 9 aa, synthetic construct
GGAGADRLE

SEQ ID NO: 397 - protein, 9 aa, synthetic construct
GGLGDDLLF

SEQ ID NO: 398 - protein, 9 aa, synthetic construct
GGAGNDRLT

SEQ ID NO: 399 - protein, 9 aa, synthetic construct
GGTGADVFR

SEQ ID NO: 400 - protein, 9 aa, synthetic construct
GGAGNDTIW

SEQ ID NO: 401 - protein, 9 aa, synthetic construct
GGLGDDILV

SEQ ID NO: 402 - protein, 9 aa, synthetic construct
GGAGSDTLI

SEQ ID NO: 403 - protein, 9 aa, synthetic construct
GGAGNDTLK

SEQ ID NO: 404 - protein, 9 aa, synthetic construct
GGGGNDTLT

SEQ ID NO: 405 - protein, 9 aa, synthetic construct
GGRGNDTLS

SEQ ID NO: 406 - protein, 9 aa, synthetic construct
GGAGADKLN

SEQ ID NO: 407 - protein, 9 aa, synthetic construct
GGEGNDLLE

SEQ ID NO: 408 - protein, 9 aa, synthetic construct
GGRGNDILL

SEQ ID NO: 409 - protein, 9 aa, synthetic construct
GGAGDDIIY

SEQ ID NO: 410 - protein, 9 aa, synthetic construct
GGNGNDLLV

SEQ ID NO: 411 - protein, 9 aa, synthetic construct
GGEGNDTLR

SEQ ID NO: 412 - protein, 9 aa, synthetic construct
GGAGDDSLD

SEQ ID NO: 413 - protein, 9 aa, synthetic construct
GGAGSDTLD

SEQ ID NO: 414 - protein, 9 aa, synthetic construct
GGEGNDILI

SEQ ID NO: 415 - protein, 9 aa, synthetic construct
GGAGGDTLT

SEQ ID NO: 416 - protein, 9 aa, synthetic construct
GGAGHDQLF

SEQ ID NO: 417 - protein, 9 aa, synthetic construct
GGLGDDTYV

SEQ ID NO: 418 - protein, 9 aa, synthetic construct
GGAGRDALY

SEQ ID NO: 419 - protein, 9 aa, synthetic construct
GGPGNDILI

SEQ ID NO: 420 - protein, 9 aa, synthetic construct
GGGGNDTII

SEQ ID NO: 421 - protein, 9 aa, synthetic construct
GGTGNDSFV

SEQ ID NO: 422 - protein, 9 aa, synthetic construct
GGAGDDVLR

SEQ ID NO: 423 - protein, 9 aa, synthetic construct
GGAGNDSLL

SEQ ID NO: 424 - protein, 9 aa, synthetic construct
GGGGADVFV

SEQ ID NO: 425 - protein, 9 aa, synthetic construct
GGTGDDTYI

SEQ ID NO: 426 - protein, 9 aa, synthetic construct
GGDGDDILY

SEQ ID NO: 427 - protein, 9 aa, synthetic construct
GGAGDDTLE

SEQ ID NO: 428 - protein, 9 aa, synthetic construct
GGAGTDTLT

SEQ ID NO: 429 - protein, 9 aa, synthetic construct
GGDGRDTLI

SEQ ID NO: 430 - protein, 9 aa, synthetic construct
GGTGADYLV

SEQ ID NO: 431 - protein, 9 aa, synthetic construct
GGAGADTID

SEQ ID NO: 432 - protein, 9 aa, synthetic construct
GGAGSDTLT

SEQ ID NO: 433 - protein, 9 aa, synthetic construct
GGEGNDTLN

SEQ ID NO: 434 - protein, 9 aa, synthetic construct
GGDGDDTLE

SEQ ID NO: 435 - protein, 9 aa, synthetic construct
GGAGRDTLI

SEQ ID NO: 436 - protein, 9 aa, synthetic construct
GGGGNDTLY

SEQ ID NO: 437 - protein, 9 aa, synthetic construct
GGLGNDILN

SEQ ID NO: 438 - protein, 9 aa, synthetic construct
GGAGNDRLV

SEQ ID NO: 439 - protein, 9 aa, synthetic construct
GGIGIDTLI

SEQ ID NO: 440 - protein, 9 aa, synthetic construct
GGVGADKLT

SEQ ID NO: 441 - protein, 9 aa, synthetic construct
GGLGADTFV

SEQ ID NO: 442 - protein, 9 aa, synthetic construct
GGDGKDLLI

SEQ ID NO: 443 - protein, 9 aa, synthetic construct
GGVGNDILI

SEQ ID NO: 444 - protein, 9 aa, synthetic construct
GGKGNDYLC

SEQ ID NO: 445 - protein, 9 aa, synthetic construct
GGAGDDTYY

SEQ ID NO: 446 - protein, 9 aa, synthetic construct
GGGGNDTIT

SEQ ID NO: 447 - protein, 9 aa, synthetic construct
GGAGKDTLT

SEQ ID NO: 448 - protein, 9 aa, synthetic construct
GGSGADTFI

SEQ ID NO: 449 - protein, 9 aa, synthetic construct
GGVGNDTLI

SEQ ID NO: 450 - protein, 9 aa, synthetic construct
GGQGNDVLI

SEQ ID NO: 451 - protein, 9 aa, synthetic construct
GGAGNDYIF

SEQ ID NO: 452 - protein, 9 aa, synthetic construct
GGAGDDTLA

SEQ ID NO: 453 - protein, 9 aa, synthetic construct
GGAGNDVID

SEQ ID NO: 454 - protein, 9 aa, synthetic construct
GGSGNDTLR

SEQ ID NO: 455 - protein, 9 aa, synthetic construct
GGDGADTLD

SEQ ID NO: 456 - protein, 9 aa, synthetic construct
GGDGADTLI

SEQ ID NO: 457 - protein, 9 aa, synthetic construct
GGAGSDTFV

SEQ ID NO: 458 - protein, 9 aa, synthetic construct
GGAGADRLV

SEQ ID NO: 459 - protein, 9 aa, synthetic construct
GGDGDDLLI

SEQ ID NO: 460 - protein, 9 aa, synthetic construct
GGDGNDILY

SEQ ID NO: 461 - protein, 9 aa, synthetic construct
GGAGADTLE

SEQ ID NO: 462 - protein, 9 aa, synthetic construct
GGAGNDDLR

SEQ ID NO: 463 - protein, 9 aa, synthetic construct
GGDGNDSLV

SEQ ID NO: 464 - protein, 9 aa, synthetic construct
GGKGNDVLD

SEQ ID NO: 465 - protein, 9 aa, synthetic construct
GGKGNDVLI

SEQ ID NO: 466 - protein, 9 aa, synthetic construct
GGGGNDTLV

SEQ ID NO: 467 - protein, 9 aa, synthetic construct
GGAGNDQLN

SEQ ID NO: 468 - protein, 9 aa, synthetic construct
GGAGSDVLN

SEQ ID NO: 469 - protein, 9 aa, synthetic construct
GGLGNDTLQ

SEQ ID NO: 470 - protein, 9 aa, synthetic construct
GGRGSDVII

SEQ ID NO: 471 - protein, 9 aa, synthetic construct
GGDGDDLLS

SEQ ID NO: 472 - protein, 9 aa, synthetic construct
GGDGNDTLR

SEQ ID NO: 473 - protein, 9 aa, synthetic construct
GGAGNDTAS

SEQ ID NO: 474 - protein, 9 aa, synthetic construct
GGPGVDEIY

SEQ ID NO: 475 - protein, 9 aa, synthetic construct
GGAGADTFI

SEQ ID NO: 476 - protein, 9 aa, synthetic construct
GGNGNDTLN

SEQ ID NO: 477 - protein, 9 aa, synthetic construct
GGGGNDTLS

SEQ ID NO: 478 - protein, 9 aa, synthetic construct
GGAGDDVLN

SEQ ID NO: 479 - protein, 9 aa, synthetic construct
GGTGDDILV

SEQ ID NO: 480 - protein, 9 aa, synthetic construct
GGAGADLLT

SEQ ID NO: 481 - protein, 9 aa, synthetic construct
GGDGNDILV

SEQ ID NO: 482 - protein, 9 aa, synthetic construct
GGNGDDWLT

SEQ ID NO: 483 - protein, 9 aa, synthetic construct
GGDGNDRLM

SEQ ID NO: 484 - protein, 9 aa, synthetic construct
GGAGADVLN

SEQ ID NO: 485 - protein, 9 aa, synthetic construct
GGDGNDTIK

SEQ ID NO: 486 - protein, 9 aa, synthetic construct
GGAGGDTLS

SEQ ID NO: 487 - protein, 9 aa, synthetic construct
GGAGNDRLL

SEQ ID NO: 488 - protein, 9 aa, synthetic construct
GGLGHDVLN

SEQ ID NO: 489 - protein, 9 aa, synthetic construct
GGAGDDSLS

SEQ ID NO: 490 - protein, 9 aa, synthetic construct
GGDGNDVLS

SEQ ID NO: 491 - protein, 9 aa, synthetic construct
GGAGNDSLF

SEQ ID NO: 492 - protein, 9 aa, synthetic construct
GGGGADTLR

SEQ ID NO: 493 - protein, 9 aa, synthetic construct
GGSGDDTLD

SEQ ID NO: 494 - protein, 9 aa, synthetic construct
GGEGDDIFK

SEQ ID NO: 495 - protein, 9 aa, synthetic construct
GGSGADTLD

SEQ ID NO: 496 - protein, 9 aa, synthetic construct
GGAGADVFD

SEQ ID NO: 497 - protein, 9 aa, synthetic construct
GGAGADKMS

SEQ ID NO: 498 - protein, 9 aa, synthetic construct
GGTGNDVFI

SEQ ID NO: 499 - protein, 9 aa, synthetic construct
GGAGNDRLA

SEQ ID NO: 500 - protein, 9 aa, synthetic construct
GGLGDDLLI

SEQ ID NO: 501 - protein, 9 aa, synthetic construct
GGAGDDVID

SEQ ID NO: 502 - protein, 9 aa, synthetic construct
GGNGNDMLF

SEQ ID NO: 503 - protein, 9 aa, synthetic construct
GGAGNDLLQ

SEQ ID NO: 504 - protein, 9 aa, synthetic construct
GGGGNDLLL

SEQ ID NO: 505 - protein, 9 aa, synthetic construct
GGDGDDTLR

SEQ ID NO: 506 - protein, 9 aa, synthetic construct
GGEGNDVLH

SEQ ID NO: 507 - protein, 9 aa, synthetic construct
GGSGNDRLE

SEQ ID NO: 508 - protein, 9 aa, synthetic construct
GGIGNDTLN

SEQ ID NO: 509 - protein, 9 aa, synthetic construct
GGAGNDTLW

SEQ ID NO: 510 - protein, 9 aa, synthetic construct
GGTGADTYV

SEQ ID NO: 511 - protein, 9 aa, synthetic construct
GGTGADTLI

SEQ ID NO: 512 - protein, 9 aa, synthetic construct
GGKGNDILI

SEQ ID NO: 513 - protein, 9 aa, synthetic construct
GGLGNDTID

SEQ ID NO: 514 - protein, 9 aa, synthetic construct
GGSGNDSLD

SEQ ID NO: 515 - protein, 9 aa, synthetic construct
GGEGKDLLI

SEQ ID NO: 516 - protein, 9 aa, synthetic construct
GGAGNDTMT

SEQ ID NO: 517 - protein, 9 aa, synthetic construct
GGSGNDILY

SEQ ID NO: 518 - protein, 9 aa, synthetic construct
GGAGRDTLS

SEQ ID NO: 519 - protein, 9 aa, synthetic construct
GGFGADTVI

SEQ ID NO: 520 - protein, 9 aa, synthetic construct
GGAGADVLI

SEQ ID NO: 521 - protein, 9 aa, synthetic construct
GGQGADIMT

SEQ ID NO: 522 - protein, 9 aa, synthetic construct
GGLGDDTYY

SEQ ID NO: 523 - protein, 9 aa, synthetic construct
GGAGSDTAD

SEQ ID NO: 524 - protein, 9 aa, synthetic construct
GGSGNDRLD

SEQ ID NO: 525 - protein, 9 aa, synthetic construct
GGDGNDKLT

SEQ ID NO: 526 - protein, 9 aa, synthetic construct
GGAGNDSLI

SEQ ID NO: 527 - protein, 9 aa, synthetic construct
GGDGADTLN

SEQ ID NO: 528 - protein, 9 aa, synthetic construct
GGLGADTLT

SEQ ID NO: 529 - protein, 9 aa, synthetic construct
GGAGVDKLT

SEQ ID NO: 530 - protein, 9 aa, synthetic construct
GGAGNDILL

SEQ ID NO: 531 - protein, 9 aa, synthetic construct
GGAGADRLS

SEQ ID NO: 532 - protein, 9 aa, synthetic construct
GGLGADTLN

SEQ ID NO: 533 - protein, 9 aa, synthetic construct
GGEGNDTLS

SEQ ID NO: 534 - protein, 9 aa, synthetic construct
GGSGNDVLI

SEQ ID NO: 535 - protein, 9 aa, synthetic construct
GGRGADFIE

SEQ ID NO: 536 - protein, 9 aa, synthetic construct
GGTGGDTLS

SEQ ID NO: 537 - protein, 9 aa, synthetic construct
GGDGNDYLY

SEQ ID NO: 538 - protein, 9 aa, synthetic construct
GGSGDDLLL

SEQ ID NO: 539 - protein, 9 aa, synthetic construct
GGTGNDTLE

SEQ ID NO: 540 - protein, 9 aa, synthetic construct
GGDGNDSLS

SEQ ID NO: 541 - protein, 9 aa, synthetic construct
GGAGNDMLS

SEQ ID NO: 542 - protein, 9 aa, synthetic construct
GGDGDDTLN

SEQ ID NO: 543 - protein, 9 aa, synthetic construct
GGDGNDVLY

SEQ ID NO: 544 - protein, 9 aa, synthetic construct
GGAGADTMT

SEQ ID NO: 545 - protein, 9 aa, synthetic construct
GGLGNDLLY

SEQ ID NO: 546 - protein, 9 aa, synthetic construct
GGSGNDILD

SEQ ID NO: 547 - protein, 9 aa, synthetic construct
GGSGNDVLY

SEQ ID NO: 548 - protein, 9 aa, synthetic construct
GGAGTDELR

SEQ ID NO: 549 - protein, 9 aa, synthetic construct
GGNGNDVMI

SEQ ID NO: 550 - protein, 9 aa, synthetic construct
GGLGNDVLD

SEQ ID NO: 551 - protein, 9 aa, synthetic construct
GGSGNDTYV

SEQ ID NO: 552 - protein, 9 aa, synthetic construct
GGKGNDSLI

SEQ ID NO: 553 - protein, 9 aa, synthetic construct
GGAGNDKLI

SEQ ID NO: 554 - protein, 9 aa, synthetic construct
GGTGDDMLY

SEQ ID NO: 555 - protein, 9 aa, synthetic construct
GGNGNDLLD

SEQ ID NO: 556 - protein, 9 aa, synthetic construct
GGTGNDLLL

SEQ ID NO: 557 - protein, 9 aa, synthetic construct
GGAGQDTLT

SEQ ID NO: 558 - protein, 9 aa, synthetic construct
GGDGNDILN

SEQ ID NO: 559 - protein, 9 aa, synthetic construct
GGAGDDILR

SEQ ID NO: 560 - protein, 9 aa, synthetic construct
GGGGNDRLD

SEQ ID NO: 561 - protein, 9 aa, synthetic construct
GGEGNDLLD

SEQ ID NO: 562 - protein, 9 aa, synthetic construct
GGAGNDYLS

SEQ ID NO: 563 - protein, 9 aa, synthetic construct
GGAGNDTIV

SEQ ID NO: 564 - protein, 9 aa, synthetic construct
GGNGVDTAD

SEQ ID NO: 565 - protein, 9 aa, synthetic construct
GGDGDDLFQ

SEQ ID NO: 566 - protein, 9 aa, synthetic construct
GGAGNDVLH

SEQ ID NO: 567 - protein, 9 aa, synthetic construct
GGLGNDTLR

SEQ ID NO: 568 - protein, 9 aa, synthetic construct
GGAGRDTLT

SEQ ID NO: 569 - protein, 9 aa, synthetic construct
GGAGNDLID

SEQ ID NO: 570 - protein, 9 aa, synthetic construct
GGDGNDLLD

SEQ ID NO: 571 - protein, 9 aa, synthetic construct
GGAGGDILV

SEQ ID NO: 572 - protein, 9 aa, synthetic construct
GGAGDDVMT

SEQ ID NO: 573 - protein, 9 aa, synthetic construct
GGDGNDTLE

SEQ ID NO: 574 - protein, 9 aa, synthetic construct
GGDGDDILD

SEQ ID NO: 575 - protein, 9 aa, synthetic construct
GGTGDDTLT

SEQ ID NO: 576 - protein, 9 aa, synthetic construct
GGDGNDVLN

SEQ ID NO: 577 - protein, 9 aa, synthetic construct
GGAGDDRLT

SEQ ID NO: 578 - protein, 9 aa, synthetic construct
GGAGDDILF

SEQ ID NO: 579 - protein, 9 aa, synthetic construct
GGAGDDRLE

SEQ ID NO: 580 - protein, 9 aa, synthetic construct
GGNGNDVLD

SEQ ID NO: 581 - protein, 9 aa, synthetic construct
GGTGIDTFD

SEQ ID NO: 582 - protein, 9 aa, synthetic construct
GGDGDDTLT

SEQ ID NO: 583 - protein, 9 aa, synthetic construct
GGAGDDRFR

SEQ ID NO: 584 - protein, 9 aa, synthetic construct
GGLGNDTYY

SEQ ID NO: 585 - protein, 9 aa, synthetic construct
GGPGNDTLT

SEQ ID NO: 586 - protein, 9 aa, synthetic construct
GGAGADRLN

SEQ ID NO: 587 - protein, 9 aa, synthetic construct
GGDGNDVIY

SEQ ID NO: 588 - protein, 9 aa, synthetic construct
GGAGRDTLD

SEQ ID NO: 589 - protein, 9 aa, synthetic construct
GGAGDDVLL

SEQ ID NO: 590 - protein, 9 aa, synthetic construct
GGAGNDQLF

SEQ ID NO: 591 - protein, 9 aa, synthetic construct
GGAGDDRLY

SEQ ID NO: 592 - protein, 9 aa, synthetic construct
GGGGADRLS

SEQ ID NO: 593 - protein, 9 aa, synthetic construct
GGDGNDLLF

SEQ ID NO: 594 - protein, 9 aa, synthetic construct
GGTGNDILD

SEQ ID NO: 595 - protein, 9 aa, synthetic construct
GGDGNDSLD

SEQ ID NO: 596 - protein, 9 aa, synthetic construct
GGAGADVLT

SEQ ID NO: 597 - protein, 9 aa, synthetic construct
GGAGNDSLV

SEQ ID NO: 598 - protein, 9 aa, synthetic construct
GGDGNDVLT

SEQ ID NO: 599 - protein, 9 aa, synthetic construct
GGAGNDRLN

SEQ ID NO: 600 - protein, 9 aa, synthetic construct
GGGGDDILI

SEQ ID NO: 601 - protein, 9 aa, synthetic construct
GGTGNDVLS

SEQ ID NO: 602 - protein, 9 aa, synthetic construct
GGDGDDLLL

SEQ ID NO: 603 - protein, 9 aa, synthetic construct
GGDGNDTIT

SEQ ID NO: 604 - protein, 9 aa, synthetic construct
GGAGVDTAD

SEQ ID NO: 605 - protein, 9 aa, synthetic construct
GGAGDDTLR

SEQ ID NO: 606 - protein, 9 aa, synthetic construct
GGAGDDTIY

SEQ ID NO: 607 - protein, 9 aa, synthetic construct
GGNGNDTLL

SEQ ID NO: 608 - protein, 9 aa, synthetic construct
GGAGVDTLT

SEQ ID NO: 609 - protein, 9 aa, synthetic construct
GGTGDDTLD

SEQ ID NO: 610 - protein, 9 aa, synthetic construct
GGNGNDTLS

SEQ ID NO: 611 - protein, 9 aa, synthetic construct
GGDGSDTAD

SEQ ID NO: 612 - protein, 9 aa, synthetic construct
GGSGNDVIY

SEQ ID NO: 613 - protein, 9 aa, synthetic construct
GGAGNDILM

SEQ ID NO: 614 - protein, 9 aa, synthetic construct
GGAGNDTLM

SEQ ID NO: 615 - protein, 9 aa, synthetic construct
GGVGNDVLK

SEQ ID NO: 616 - protein, 9 aa, synthetic construct
GGDGNDSLY

SEQ ID NO: 617 - protein, 9 aa, synthetic construct
GGAGADVII

SEQ ID NO: 618 - protein, 9 aa, synthetic construct
GGIGNDTLD

SEQ ID NO: 619 - protein, 9 aa, synthetic construct
GGDGDDVID

SEQ ID NO: 620 - protein, 9 aa, synthetic construct
GGKGNDYLD

SEQ ID NO: 621 - protein, 9 aa, synthetic construct
GGLGDDILD

SEQ ID NO: 622 - protein, 9 aa, synthetic construct
GGDGNDRLD

SEQ ID NO: 623 - protein, 9 aa, synthetic construct
GGAGNDTIS

SEQ ID NO: 624 - protein, 9 aa, synthetic construct
GGEGNDILK

SEQ ID NO: 625 - protein, 9 aa, synthetic construct
GGEGNDRLD

SEQ ID NO: 626 - protein, 9 aa, synthetic construct
GGTGNDYLS

SEQ ID NO: 627 - protein, 9 aa, synthetic construct
GGAGNDYLV

SEQ ID NO: 628 - protein, 9 aa, synthetic construct
GGEGADTFV

SEQ ID NO: 629 - protein, 9 aa, synthetic construct
GGLGADTMI

SEQ ID NO: 630 - protein, 9 aa, synthetic construct
GGWGNDTLN

SEQ ID NO: 631 - protein, 9 aa, synthetic construct
GGAGADILT

SEQ ID NO: 632 - protein, 9 aa, synthetic construct
GGAGADSLT

SEQ ID NO: 633 - protein, 9 aa, synthetic construct
GGSGNDRLI

SEQ ID NO: 634 - protein, 9 aa, synthetic construct
GGSGNDILR

SEQ ID NO: 635 - protein, 9 aa, synthetic construct
GGSGGDTFV

SEQ ID NO: 636 - protein, 9 aa, synthetic construct
GGGGNDTID

SEQ ID NO: 637 - protein, 9 aa, synthetic construct
GGVGKDTLY

SEQ ID NO: 638 - protein, 9 aa, synthetic construct
GGLGNDYLQ

SEQ ID NO: 639 - protein, 9 aa, synthetic construct
GGSGNDRLY

SEQ ID NO: 640 - protein, 9 aa, synthetic construct
GGAGVDTLI

SEQ ID NO: 641 - protein, 9 aa, synthetic construct
GGEGNDLLF

SEQ ID NO: 642 - protein, 9 aa, synthetic construct
GGIGNDRLF

SEQ ID NO: 643 - protein, 9 aa, synthetic construct
GGAGIDTAS

SEQ ID NO: 644 - protein, 9 aa, synthetic construct
GGDGNDRLL

SEQ ID NO: 645 - protein, 9 aa, synthetic construct
GGAGDDYLD

SEQ ID NO: 646 - protein, 9 aa, synthetic construct
GGLGDDVLR

SEQ ID NO: 647 - protein, 9 aa, synthetic construct
GGSGNDTLA

SEQ ID NO: 648 - protein, 9 aa, synthetic construct
GGDGRDTLL

SEQ ID NO: 649 - protein, 9 aa, synthetic construct
GGAGDDVLE

SEQ ID NO: 650 - protein, 9 aa, synthetic construct
GGTGNDTLV

SEQ ID NO: 651 - protein, 9 aa, synthetic construct
GGTGNDSLD

SEQ ID NO: 652 - protein, 9 aa, synthetic construct
GGTGADRFV

SEQ ID NO: 653 - protein, 9 aa, synthetic construct
GGSGNDYLS

SEQ ID NO: 654 - protein, 9 aa, synthetic construct
GGAGDDFLD

SEQ ID NO: 655 - protein, 9 aa, synthetic construct
GGVGIDKME

SEQ ID NO: 656 - protein, 9 aa, synthetic construct
GGAGTDWLK

SEQ ID NO: 657 - protein, 9 aa, synthetic construct
GGGGDDLLS

SEQ ID NO: 658 - protein, 9 aa, synthetic construct
GGGGDDVLS

SEQ ID NO: 659 - protein, 9 aa, synthetic construct
GGSGNDRLF

SEQ ID NO: 660 - protein, 9 aa, synthetic construct
GGAGNDELR

SEQ ID NO: 661 - protein, 9 aa, synthetic construct
GGQGNDVFV

SEQ ID NO: 662 - protein, 9 aa, synthetic construct
GGAGNDELN

SEQ ID NO: 663 - protein, 9 aa, synthetic construct
GGAGNDKLD

SEQ ID NO: 664 - protein, 9 aa, synthetic construct
GGAGNDGLL

SEQ ID NO: 665 - protein, 9 aa, synthetic construct
GGAGDDLLS

SEQ ID NO: 666 - protein, 9 aa, synthetic construct
GGAGNDQLD

SEQ ID NO: 667 - protein, 9 aa, synthetic construct
GGAGSDTLN

SEQ ID NO: 668 - protein, 9 aa, synthetic construct
GGAGADRLY

SEQ ID NO: 669 - protein, 9 aa, synthetic construct
GGKGDDTYI

SEQ ID NO: 670 - protein, 9 aa, synthetic construct
GGDGDDSLD

SEQ ID NO: 671 - protein, 9 aa, synthetic construct
GGLGKDVLD

SEQ ID NO: 672 - protein, 9 aa, synthetic construct
GGIGDDILI

SEQ ID NO: 673 - protein, 9 aa, synthetic construct
GGKGNDYLN

SEQ ID NO: 674 - protein, 9 aa, synthetic construct
GGAGSDTLV

SEQ ID NO: 675 - protein, 9 aa, synthetic construct
GGGGDDSFK

SEQ ID NO: 676 - protein, 9 aa, synthetic construct
GGAGDDIIT

SEQ ID NO: 677 - protein, 9 aa, synthetic construct
GGLGDDTLI

SEQ ID NO: 678 - protein, 9 aa, synthetic construct
GGTGNDKLY

SEQ ID NO: 679 - protein, 9 aa, synthetic construct
GGAGNDTIF

SEQ ID NO: 680 - protein, 9 aa, synthetic construct
GGLGNDVMR

SEQ ID NO: 681 - protein, 9 aa, synthetic construct
GGQGNDVLV

SEQ ID NO: 682 - protein, 9 aa, synthetic construct
GGSGDDTLL

SEQ ID NO: 683 - protein, 9 aa, synthetic construct
GGAGIDTVV

SEQ ID NO: 684 - protein, 9 aa, synthetic construct
GGAGADTLF

SEQ ID NO: 685 - protein, 9 aa, synthetic construct
GGAGADDII

SEQ ID NO: 686 - protein, 9 aa, synthetic construct
GGLGNDTLY

SEQ ID NO: 687 - protein, 9 aa, synthetic construct
GGSGNDSLI

SEQ ID NO: 688 - protein, 9 aa, synthetic construct
GGAGNDVLQ

SEQ ID NO: 689 - protein, 9 aa, synthetic construct
GGDGADTLS

SEQ ID NO: 690 - protein, 9 aa, synthetic construct
GGAGRDTFV

SEQ ID NO: 691 - protein, 9 aa, synthetic construct
GGGGADRLR

SEQ ID NO: 692 - protein, 9 aa, synthetic construct
GGAGEDTLI

SEQ ID NO: 693 - protein, 9 aa, synthetic construct
GGQGVDTFS

SEQ ID NO: 694 - protein, 9 aa, synthetic construct
GGQGNDTLY

SEQ ID NO: 695 - protein, 9 aa, synthetic construct
GGQGNDTLN

SEQ ID NO: 696 - protein, 9 aa, synthetic construct
GGKGADTLD

SEQ ID NO: 697 - protein, 9 aa, synthetic construct
GGVGADTLT

SEQ ID NO: 698 - protein, 9 aa, synthetic construct
GGEGNDTLY

SEQ ID NO: 699 - protein, 9 aa, synthetic construct
GGDGNDVLH

SEQ ID NO: 700 - protein, 9 aa, synthetic construct
GGDGNDILD

SEQ ID NO: 701 - protein, 9 aa, synthetic construct
GGTGNDILR

SEQ ID NO: 702 - protein, 9 aa, synthetic construct
GGTGNDLLD

SEQ ID NO: 703 - protein, 9 aa, synthetic construct
GGDGNDVLL

SEQ ID NO: 704 - protein, 9 aa, synthetic construct
GGSGADIMR

SEQ ID NO: 705 - protein, 9 aa, synthetic construct
GGAGDDILS

SEQ ID NO: 706 - protein, 9 aa, synthetic construct
GGGGDDTLI

SEQ ID NO: 707 - protein, 9 aa, synthetic construct
GGAGADSLS

SEQ ID NO: 708 - protein, 9 aa, synthetic construct
GGSGNDLLD

SEQ ID NO: 709 - protein, 9 aa, synthetic construct
GGGGSDILF

SEQ ID NO: 710 - protein, 9 aa, synthetic construct
GGVGNDVYI

SEQ ID NO: 711 - protein, 9 aa, synthetic construct
GGDGNDLLV

SEQ ID NO: 712 - protein, 9 aa, synthetic construct
GGDGNDVLF

SEQ ID NO: 713 - protein, 9 aa, synthetic construct
GGAGNDSID

SEQ ID NO: 714 - protein, 9 aa, synthetic construct
GGDGNDFLA

SEQ ID NO: 715 - protein, 9 aa, synthetic construct
GGAGNDALN

SEQ ID NO: 716 - protein, 9 aa, synthetic construct
GGAGEDVLR

SEQ ID NO: 717 - protein, 9 aa, synthetic construct
GGTGNDTYR

SEQ ID NO: 718 - protein, 9 aa, synthetic construct
GGDGDDYLD

SEQ ID NO: 719 - protein, 9 aa, synthetic construct
GGEGNDTLQ

SEQ ID NO: 720 - protein, 9 aa, synthetic construct
GGEGNDSLD

SEQ ID NO: 721 - protein, 9 aa, synthetic construct
GGTGNDVYY

SEQ ID NO: 722 - protein, 9 aa, synthetic construct
GGIGEDTFI

SEQ ID NO: 723 - protein, 9 aa, synthetic construct
GGEGNDTLV

SEQ ID NO: 724 - protein, 9 aa, synthetic construct
GGDGSDTFK

SEQ ID NO: 725 - protein, 9 aa, synthetic construct
GGAGDDVLF

SEQ ID NO: 726 - protein, 9 aa, synthetic construct
GGNGKDILK

SEQ ID NO: 727 - protein, 9 aa, synthetic construct
GGTGADTLT

SEQ ID NO: 728 - protein, 9 aa, synthetic construct
GGEGNDILL

SEQ ID NO: 729 - protein, 9 aa, synthetic construct
GGAGADILI

SEQ ID NO: 730 - protein, 9 aa, synthetic construct
GGAGNDIYR

SEQ ID NO: 731 - protein, 9 aa, synthetic construct
GGAGNDLLT

SEQ ID NO: 732 - protein, 9 aa, synthetic construct
GGKGNDLLH

SEQ ID NO: 733 - protein, 9 aa, synthetic construct
GGKGNDLLI

SEQ ID NO: 734 - protein, 9 aa, synthetic construct
GGSGADTLT

SEQ ID NO: 735 - protein, 9 aa, synthetic construct
GGDGNDQIF

SEQ ID NO: 736 - protein, 9 aa, synthetic construct
GGEGDDILI

SEQ ID NO: 737 - protein, 9 aa, synthetic construct
GGTGDDTYV

SEQ ID NO: 738 - protein, 9 aa, synthetic construct
GGVGADTLV

SEQ ID NO: 739 - protein, 9 aa, synthetic construct
GGKGNDRLV

SEQ ID NO: 740 - protein, 9 aa, synthetic construct
GGDGNDTIY

SEQ ID NO: 741 - protein, 9 aa, synthetic construct
GGDGNDTIL

SEQ ID NO: 742 - protein, 9 aa, synthetic construct
GGTGNDYLE

SEQ ID NO: 743 - protein, 9 aa, synthetic construct
GGAGNDIYV

SEQ ID NO: 744 - protein, 9 aa, synthetic construct
GGLGIDRLT

SEQ ID NO: 745 - protein, 9 aa, synthetic construct
GGDGDDYID

SEQ ID NO: 746 - protein, 9 aa, synthetic construct
GGEGDDLLK

SEQ ID NO: 747 - protein, 9 aa, synthetic construct
GGAGDDKLT

SEQ ID NO: 748 - protein, 9 aa, synthetic construct
GGAGADKLY

SEQ ID NO: 749 - protein, 9 aa, synthetic construct
GGQGEDSLR

SEQ ID NO: 750 - protein, 9 aa, synthetic construct
GGTGNDTLA

SEQ ID NO: 751 - protein, 9 aa, synthetic construct
GGAGLDTLI

SEQ ID NO: 752 - protein, 9 aa, synthetic construct
GGAGDDRLN

SEQ ID NO: 753 - protein, 9 aa, synthetic construct
GGAGADEIY

SEQ ID NO: 754 - protein, 9 aa, synthetic construct
GGAGNDQLY

SEQ ID NO: 755 - protein, 9 aa, synthetic construct
GGDGNDTLF

SEQ ID NO: 756 - protein, 9 aa, synthetic construct
GGAGKDTLY

SEQ ID NO: 757 - protein, 9 aa, synthetic construct
GGGGADVLW

SEQ ID NO: 758 - protein, 9 aa, synthetic construct
GGAGDDTLF

SEQ ID NO: 759 - protein, 9 aa, synthetic construct
GGGGDDIFS

SEQ ID NO: 760 - protein, 9 aa, synthetic construct
GGAGDDTLQ

SEQ ID NO: 761 - protein, 9 aa, synthetic construct
GGGGNDVLI

SEQ ID NO: 762 - protein, 9 aa, synthetic construct
GGIGNDKLF

SEQ ID NO: 763 - protein, 9 aa, synthetic construct
GGAGIDTAD

SEQ ID NO: 764 - protein, 9 aa, synthetic construct
GGLGADTMT

SEQ ID NO: 765 - protein, 9 aa, synthetic construct
GGLGDDTLN

SEQ ID NO: 766 - protein, 9 aa, synthetic construct
GGDGDDYIE

SEQ ID NO: 767 - protein, 9 aa, synthetic construct
GGEGDDTLI

SEQ ID NO: 768 - protein, 9 aa, synthetic construct
GGDGNDALY

SEQ ID NO: 769 - protein, 9 aa, synthetic construct
GGKGDDIFV

SEQ ID NO: 770 - protein, 9 aa, synthetic construct
GGNGDDTLI

SEQ ID NO: 771 - protein, 9 aa, synthetic construct
GGSGNDTID

SEQ ID NO: 772 - protein, 9 aa, synthetic construct
GGSGNDNLY

SEQ ID NO: 773 - protein, 9 aa, synthetic construct
GGEGDDQVI

SEQ ID NO: 774 - protein, 9 aa, synthetic construct
GGLGDDILY

SEQ ID NO: 775 - protein, 9 aa, synthetic construct
GGAGNDLLF

SEQ ID NO: 776 - protein, 9 aa, synthetic construct
GGTGDDTLN

SEQ ID NO: 777 - protein, 9 aa, synthetic construct
GGTGNDLLK

SEQ ID NO: 778 - protein, 9 aa, synthetic construct
GGSGNDILN

SEQ ID NO: 779 - protein, 9 aa, synthetic construct
GGAGNDILW

SEQ ID NO: 780 - protein, 9 aa, synthetic construct
GGAGNDALS

SEQ ID NO: 781 - protein, 9 aa, synthetic construct
GGAGDDELN

SEQ ID NO: 782 - protein, 9 aa, synthetic construct
GGEGNDILV

SEQ ID NO: 783 - protein, 9 aa, synthetic construct
GGLGDDLLD

SEQ ID NO: 784 - protein, 9 aa, synthetic construct
GGDGDDRLD

SEQ ID NO: 785 - protein, 9 aa, synthetic construct
GGGGNDFIN

SEQ ID NO: 786 - protein, 9 aa, synthetic construct
GGDGDDLID

SEQ ID NO: 787 - protein, 9 aa, synthetic construct
GGAGADILD

SEQ ID NO: 788 - protein, 9 aa, synthetic construct
GGSGNDYLA

SEQ ID NO: 789 - protein, 9 aa, synthetic construct
GGDGDDTLV

SEQ ID NO: 790 - protein, 9 aa, synthetic construct
GGAGADRLL

SEQ ID NO: 791 - protein, 9 aa, synthetic construct
GGAGTDTAS

SEQ ID NO: 792 - protein, 9 aa, synthetic construct
GGDGNDILR

SEQ ID NO: 793 - protein, 9 aa, synthetic construct
GGDGDDLIY

SEQ ID NO: 794 - protein, 9 aa, synthetic construct
GGAGDDQLF

SEQ ID NO: 795 - protein, 9 aa, synthetic construct
GGAGRDALS

SEQ ID NO: 796 - protein, 9 aa, synthetic construct
GGAGSDRLT

SEQ ID NO: 797 - protein, 9 aa, synthetic construct
GGTGDDVLY

SEQ ID NO: 798 - protein, 9 aa, synthetic construct
GGDGNDTVF

SEQ ID NO: 799 - protein, 9 aa, synthetic construct
GGSGIDTLI

SEQ ID NO: 800 - protein, 9 aa, synthetic construct
GGNGNDQLY

SEQ ID NO: 801 - protein, 9 aa, synthetic construct
GGAGADHFV

SEQ ID NO: 802 - protein, 9 aa, synthetic construct
GGSGDDVLI

SEQ ID NO: 803 - protein, 9 aa, synthetic construct
GGIGDDTLS

SEQ ID NO: 804 - protein, 9 aa, synthetic construct
GGEGDDSIL

SEQ ID NO: 805 - protein, 9 aa, synthetic construct
GGDGIDILI

SEQ ID NO: 806 - protein, 9 aa, synthetic construct
GGEGNDTID

SEQ ID NO: 807 - protein, 9 aa, synthetic construct
GGSGDDRLF

SEQ ID NO: 808 - protein, 9 aa, synthetic construct
GGSGNDILV

SEQ ID NO: 809 - protein, 9 aa, synthetic construct
GGVGNDTLY

SEQ ID NO: 810 - protein, 9 aa, synthetic construct
GGAGADALD

SEQ ID NO: 811 - protein, 9 aa, synthetic construct
GGGGSDTAD

SEQ ID NO: 812 - protein, 9 aa, synthetic construct
GGDGNDSID

SEQ ID NO: 813 - protein, 9 aa, synthetic construct
GGSGTDHLW

SEQ ID NO: 814 - protein, 9 aa, synthetic construct
GGTGDDTLI

SEQ ID NO: 815 - protein, 9 aa, synthetic construct
GGDGNDILT

SEQ ID NO: 816 - protein, 9 aa, synthetic construct
GGAGNDLIM

SEQ ID NO: 817 - protein, 9 aa, synthetic construct
GGLGDDTYI

SEQ ID NO: 818 - protein, 9 aa, synthetic construct
GGAGNDVLA

SEQ ID NO: 819 - protein, 9 aa, synthetic construct
GGAGGDVIN

SEQ ID NO: 820 - protein, 9 aa, synthetic construct
GGAGDDVIL

SEQ ID NO: 821 - protein, 9 aa, synthetic construct
GGSGQDYLD

SEQ ID NO: 822 - protein, 9 aa, synthetic construct
GGAGNDVIN

SEQ ID NO: 823 - protein, 9 aa, synthetic construct
GGIGNDTLI

SEQ ID NO: 824 - protein, 9 aa, synthetic construct
GGAGNDWLD

SEQ ID NO: 825 - protein, 9 aa, synthetic construct
GGAGNDSIT

SEQ ID NO: 826 - protein, 9 aa, synthetic construct
GGAGNDSYV

SEQ ID NO: 827 - protein, 9 aa, synthetic construct
GGTGNDILI

SEQ ID NO: 828 - protein, 9 aa, synthetic construct
GGAGDDMLD

SEQ ID NO: 829 - protein, 9 aa, synthetic construct
GGTGNDTLK

SEQ ID NO: 830 - protein, 9 aa, synthetic construct
GGLGDDVIE

SEQ ID NO: 831 - protein, 9 aa, synthetic construct
GGLGDDTLT

SEQ ID NO: 832 - protein, 9 aa, synthetic construct
GGAGADRLF

SEQ ID NO: 833 - protein, 9 aa, synthetic construct
GGYGNDILT

SEQ ID NO: 834 - protein, 9 aa, synthetic construct
GGAGNDLLL

SEQ ID NO: 835 - protein, 9 aa, synthetic construct
GGSGADVFV

SEQ ID NO: 836 - protein, 9 aa, synthetic construct
GGNGDDILN

SEQ ID NO: 837 - protein, 9 aa, synthetic construct
GGGGRDTLW

SEQ ID NO: 838 - protein, 9 aa, synthetic construct
GGGGADTLL

SEQ ID NO: 839 - protein, 9 aa, synthetic construct
GGKGNDTYV

SEQ ID NO: 840 - protein, 9 aa, synthetic construct
GGAGDDTIN

SEQ ID NO: 841 - protein, 9 aa, synthetic construct
GGLGNDVLI

SEQ ID NO: 842 - protein, 9 aa, synthetic construct
GGQGDDILY

SEQ ID NO: 843 - protein, 9 aa, synthetic construct
GGVGNDTLT

SEQ ID NO: 844 - protein, 9 aa, synthetic construct
GGDGNDLLS

SEQ ID NO: 845 - protein, 9 aa, synthetic construct
GGAGDDEIS

SEQ ID NO: 846 - protein, 9 aa, synthetic construct
GGGGADTYD

SEQ ID NO: 847 - protein, 9 aa, synthetic construct
GGLGNDVLR

SEQ ID NO: 848 - protein, 9 aa, synthetic construct
GGGGADRLY

SEQ ID NO: 849 - protein, 9 aa, synthetic construct
GGAGDDTYL

SEQ ID NO: 850 - protein, 9 aa, synthetic construct
GGAGNDNLY

SEQ ID NO: 851 - protein, 9 aa, synthetic construct
GGSGDDLLI

SEQ ID NO: 852 - protein, 9 aa, synthetic construct
GGLGNDQLS

SEQ ID NO: 853 - protein, 9 aa, synthetic construct
GGTGNDVLT

SEQ ID NO: 854 - protein, 9 aa, synthetic construct
GGSGNDVLE

SEQ ID NO: 855 - protein, 9 aa, synthetic construct
GGAGADYLD

SEQ ID NO: 856 - protein, 9 aa, synthetic construct
GGGGDDVLI

SEQ ID NO: 857 - protein, 9 aa, synthetic construct
GGDGNDVLV

SEQ ID NO: 858 - protein, 9 aa, synthetic construct
GGSGDDTIY

SEQ ID NO: 859 - protein, 9 aa, synthetic construct
GGAGNDIYY

SEQ ID NO: 860 - protein, 9 aa, synthetic construct
GGNGDDTLD

SEQ ID NO: 861 - protein, 9 aa, synthetic construct
GGRGNDLLI

SEQ ID NO: 862 - protein, 9 aa, synthetic construct
GGGGTDLIR

SEQ ID NO: 863 - protein, 9 aa, synthetic construct
GGAGNDSIS

SEQ ID NO: 864 - protein, 9 aa, synthetic construct
GGAGDDTFV

SEQ ID NO: 865 - protein, 9 aa, synthetic construct
GGNGNDLLY

SEQ ID NO: 866 - protein, 9 aa, synthetic construct
GGVGNDVIK

SEQ ID NO: 867 - protein, 9 aa, synthetic construct
GGEGADTLD

SEQ ID NO: 868 - protein, 9 aa, synthetic construct
GGKGNDTYI

SEQ ID NO: 869 - protein, 9 aa, synthetic construct
GGSGNDILT

SEQ ID NO: 870 - protein, 9 aa, synthetic construct
GGSGDDVLD

SEQ ID NO: 871 - protein, 9 aa, synthetic construct
GGAGNDELY

SEQ ID NO: 872 - protein, 9 aa, synthetic construct
GGAGDDLLN

SEQ ID NO: 873 - protein, 9 aa, synthetic construct
GGGGDDLLF

SEQ ID NO: 874 - protein, 9 aa, synthetic construct
GGDGDDYLE

SEQ ID NO: 875 - protein, 9 aa, synthetic construct
GGEGADTLI

SEQ ID NO: 876 - protein, 9 aa, synthetic construct
GGYGNDTLD

SEQ ID NO: 877 - protein, 9 aa, synthetic construct
GGKGNDQLK

SEQ ID NO: 878 - protein, 9 aa, synthetic construct
GGDGNDNLA

SEQ ID NO: 879 - protein, 9 aa, synthetic construct
GGDGNDTLA

SEQ ID NO: 880 - protein, 9 aa, synthetic construct
GGTGSDTMR

SEQ ID NO: 881 - protein, 9 aa, synthetic construct
GGLGNDLLD

SEQ ID NO: 882 - protein, 9 aa, synthetic construct
GGNGNDRLY

SEQ ID NO: 883 - protein, 9 aa, synthetic construct
GGGGNDILV

SEQ ID NO: 884 - protein, 9 aa, synthetic construct
GGGGADTLW

SEQ ID NO: 885 - protein, 9 aa, synthetic construct
GGFGNDRMW

SEQ ID NO: 886 - protein, 9 aa, synthetic construct
GGNGNDSMY

SEQ ID NO: 887 - protein, 9 aa, synthetic construct
GGLGADILT

SEQ ID NO: 888 - protein, 9 aa, synthetic construct
GGDGADFVS

SEQ ID NO: 889 - protein, 9 aa, synthetic construct
GGTGNDRLL

SEQ ID NO: 890 - protein, 9 aa, synthetic construct
GGKGNDILR

SEQ ID NO: 891 - protein, 9 aa, synthetic construct
GGNGDDLLD

SEQ ID NO: 892 - protein, 9 aa, synthetic construct
GGLGNDKLF

SEQ ID NO: 893 - protein, 9 aa, synthetic construct
GGAGSDTMS

SEQ ID NO: 894 - protein, 9 aa, synthetic construct
GGSGQDTLT

SEQ ID NO: 895 - protein, 9 aa, synthetic construct
GGSGNDVLN

SEQ ID NO: 896 - protein, 9 aa, synthetic construct
GGSGNDTIN

SEQ ID NO: 897 - protein, 9 aa, synthetic construct
GGDGLDVIW

SEQ ID NO: 898 - protein, 9 aa, synthetic construct
GGNGDDFID

SEQ ID NO: 899 - protein, 9 aa, synthetic construct
GGIGADTAI

SEQ ID NO: 900 - protein, 9 aa, synthetic construct
GGAGADQLI

SEQ ID NO: 901 - protein, 9 aa, synthetic construct
GGAGNDMLY

SEQ ID NO: 902 - protein, 9 aa, synthetic construct
GGKGADQMS

SEQ ID NO: 903 - protein, 9 aa, synthetic construct
GGGGNDRLE

SEQ ID NO: 904 - protein, 9 aa, synthetic construct
GGGGNDLLD

SEQ ID NO: 905 - protein, 9 aa, synthetic construct
GGLGADTLS

SEQ ID NO: 906 - protein, 9 aa, synthetic construct
GGAGNDVLW

SEQ ID NO: 907 - protein, 9 aa, synthetic construct
GGHGDDILI

SEQ ID NO: 908 - protein, 9 aa, synthetic construct
GGDGDDRLE

SEQ ID NO: 909 - protein, 9 aa, synthetic construct
GGEGNDTLT

SEQ ID NO: 910 - protein, 9 aa, synthetic construct
GGDGNDRLE

SEQ ID NO: 911 - protein, 9 aa, synthetic construct
GGAGDDMIE

SEQ ID NO: 912 - protein, 9 aa, synthetic construct
GGAGNDALY

SEQ ID NO: 913 - protein, 9 aa, synthetic construct
GGLGDDTLS

SEQ ID NO: 914 - protein, 9 aa, synthetic construct
GGEGDDTLV

SEQ ID NO: 915 - protein, 9 aa, synthetic construct
GGLGDDTLD

SEQ ID NO: 916 - protein, 9 aa, synthetic construct
GGAGADTAD

SEQ ID NO: 917 - protein, 9 aa, synthetic construct
GGTGNDTLR

SEQ ID NO: 918 - protein, 9 aa, synthetic construct
GGAGDDALR

SEQ ID NO: 919 - protein, 9 aa, synthetic construct
GGIGDDTLI

SEQ ID NO: 920 - protein, 9 aa, synthetic construct
GGEGNDRLF

SEQ ID NO: 921 - protein, 9 aa, synthetic construct
GGNGNDSLV

SEQ ID NO: 922 - protein, 9 aa, synthetic construct
GGLGDDVLY

SEQ ID NO: 923 - protein, 9 aa, synthetic construct
GGNGDDVLE

SEQ ID NO: 924 - protein, 9 aa, synthetic construct
GGTGNDVLY

SEQ ID NO: 925 - protein, 9 aa, synthetic construct
GGLGADNLW

SEQ ID NO: 926 - protein, 9 aa, synthetic construct
GGGGGDSLW

SEQ ID NO: 927 - protein, 9 aa, synthetic construct
GGAGTDTAV

SEQ ID NO: 928 - protein, 9 aa, synthetic construct
GGGGNDVLN

SEQ ID NO: 929 - protein, 9 aa, synthetic construct
GGAGNDVLK

SEQ ID NO: 930 - protein, 9 aa, synthetic construct
GGSGNDTYL

SEQ ID NO: 931 - protein, 9 aa, synthetic construct
GGEGDDTLT

SEQ ID NO: 932 - protein, 9 aa, synthetic construct
GGLGNDTLL

SEQ ID NO: 933 - protein, 9 aa, synthetic construct
GGAGNDIIF

SEQ ID NO: 934 - protein, 9 aa, synthetic construct
GGLGNDRLY

SEQ ID NO: 935 - protein, 9 aa, synthetic construct
GGDGADTLT

SEQ ID NO: 936 - protein, 9 aa, synthetic construct
GGDGDDTID

SEQ ID NO: 937 - protein, 9 aa, synthetic construct
GGAGDDVIN

SEQ ID NO: 938 - protein, 9 aa, synthetic construct
GGGGNDTLR

SEQ ID NO: 939 - protein, 9 aa, synthetic construct
GGRGNDTIL

SEQ ID NO: 940 - protein, 9 aa, synthetic construct
GGNGADRLI

SEQ ID NO: 941 - protein, 9 aa, synthetic construct
GGDGNDTIF

SEQ ID NO: 942 - protein, 9 aa, synthetic construct
GGLGNDSLT

SEQ ID NO: 943 - protein, 9 aa, synthetic construct
GGIGNDKLY

SEQ ID NO: 944 - protein, 9 aa, synthetic construct
GGAGDDRLS

SEQ ID NO: 945 - protein, 9 aa, synthetic construct
GGEGNDVYL

SEQ ID NO: 946 - protein, 9 aa, synthetic construct
GGAGNDTVI

SEQ ID NO: 947 - protein, 9 aa, synthetic construct
GGDGADTLL

SEQ ID NO: 948 - protein, 9 aa, synthetic construct
GGKGNDTYT

SEQ ID NO: 949 - protein, 9 aa, synthetic construct
GGAGRDRLT

SEQ ID NO: 950 - protein, 9 aa, synthetic construct
GGPGNDTLS

SEQ ID NO: 951 - protein, 9 aa, synthetic construct
GGSGNDSLY

SEQ ID NO: 952 - protein, 9 aa, synthetic construct
GGDGNDSLL

SEQ ID NO: 953 - protein, 9 aa, synthetic construct
GGAGDDLLE

SEQ ID NO: 954 - protein, 9 aa, synthetic construct
GGDGNDTLQ

SEQ ID NO: 955 - protein, 9 aa, synthetic construct
GGMGEDIMT

SEQ ID NO: 956 - protein, 9 aa, synthetic construct
GGAGDDLLF

SEQ ID NO: 957 - protein, 9 aa, synthetic construct
GGAGNDSIY

SEQ ID NO: 958 - protein, 9 aa, synthetic construct
GGNGNDILD

SEQ ID NO: 959 - protein, 9 aa, synthetic construct
GGAGDDTLH

SEQ ID NO: 960 - protein, 9 aa, synthetic construct
GGEGNDSLY

SEQ ID NO: 961 - protein, 9 aa, synthetic construct
GGGGNDTLE

SEQ ID NO: 962 - protein, 9 aa, synthetic construct
GGDGDDRLN

SEQ ID NO: 963 - protein, 9 aa, synthetic construct
GGLGNDVID

SEQ ID NO: 964 - protein, 9 aa, synthetic construct
GGAGADTIT

SEQ ID NO: 965 - protein, 9 aa, synthetic construct
GGEGNDRYE

SEQ ID NO: 966 - protein, 9 aa, synthetic construct
GGIGNDTYV

SEQ ID NO: 967 - protein, 9 aa, synthetic construct
GGLGNDILD

SEQ ID NO: 968 - protein, 9 aa, synthetic construct
GGEGNDTLE

SEQ ID NO: 969 - protein, 9 aa, synthetic construct
GGKGADKLH

SEQ ID NO: 970 - protein, 9 aa, synthetic construct
GGAGNDMLD

SEQ ID NO: 971 - protein, 9 aa, synthetic construct
GGLGNDSLD

SEQ ID NO: 972 - protein, 9 aa, synthetic construct
GGKGDDTLT

SEQ ID NO: 973 - protein, 9 aa, synthetic construct
GGSGNDLLI

SEQ ID NO: 974 - protein, 9 aa, synthetic construct
GGHGNDTVF

SEQ ID NO: 975 - protein, 9 aa, synthetic construct
GGKGDDTMT

SEQ ID NO: 976 - protein, 9 aa, synthetic construct
GGGGNDILY

SEQ ID NO: 977 - protein, 9 aa, synthetic construct
GGVGTDTLT

SEQ ID NO: 978 - protein, 9 aa, synthetic construct
GGRGNDSLT

SEQ ID NO: 979 - protein, 9 aa, synthetic construct
GGGGNDVII

SEQ ID NO: 980 - protein, 9 aa, synthetic construct
GGLGDDLYF

SEQ ID NO: 981 - protein, 9 aa, synthetic construct
GGAGSDDMR

SEQ ID NO: 982 - protein, 9 aa, synthetic construct
GGTGNDVFV

SEQ ID NO: 983 - protein, 9 aa, synthetic construct
GGVGNDYLE

SEQ ID NO: 984 - protein, 9 aa, synthetic construct
GGEGDDRLY

SEQ ID NO: 985 - protein, 9 aa, synthetic construct
GGTGDDTVV

SEQ ID NO: 986 - protein, 9 aa, synthetic construct
GGDGDDVLT

SEQ ID NO: 987 - protein, 9 aa, synthetic construct
GGDGDDTLA

SEQ ID NO: 988 - protein, 9 aa, synthetic construct
GGDGADLVC

SEQ ID NO: 989 - protein, 9 aa, synthetic construct
GGAGSDELH

SEQ ID NO: 990 - protein, 9 aa, synthetic construct
GGGGHDTLT

SEQ ID NO: 991 - protein, 9 aa, synthetic construct
GGNGNDTLW

SEQ ID NO: 992 - protein, 9 aa, synthetic construct
GGKGVDFIE

SEQ ID NO: 993 - protein, 9 aa, synthetic construct
GGSGNDTIY

SEQ ID NO: 994 - protein, 9 aa, synthetic construct
GGGGDDFLI

SEQ ID NO: 995 - protein, 9 aa, synthetic construct
GGTGADTLD

SEQ ID NO: 996 - protein, 9 aa, synthetic construct
GGDGDDSID

SEQ ID NO: 997 - protein, 9 aa, synthetic construct
GGEGKDLYI

SEQ ID NO: 998 - protein, 9 aa, synthetic construct
GGEGNDTYI

SEQ ID NO: 999 - protein, 9 aa, synthetic construct
GGEGDDTLL

SEQ ID NO: 1000 - protein, 9 aa, synthetic construct
GGKGDDIID

SEQ ID NO: 1001 - protein, 9 aa, synthetic construct
GGAGADTMS

SEQ ID NO: 1002 - protein, 9 aa, synthetic construct
GGTGNDVLN

SEQ ID NO: 1003 - protein, 9 aa, synthetic construct
GGAGADTLQ

SEQ ID NO: 1004 - protein, 9 aa, synthetic construct
GGEGNDTLH

SEQ ID NO: 1005 - protein, 9 aa, synthetic construct
GGSGADQFI

SEQ ID NO: 1006 - protein, 9 aa, synthetic construct
GGLGSDTYQ

SEQ ID NO: 1007 - protein, 9 aa, synthetic construct
GGAGKDIMT

SEQ ID NO: 1008 - protein, 9 aa, synthetic construct
GGAGNDVLE

SEQ ID NO: 1009 - protein, 9 aa, synthetic construct
GGAGDDTIE

SEQ ID NO: 1010 - protein, 9 aa, synthetic construct
GGDGDDVLF

SEQ ID NO: 1011 - protein, 9 aa, synthetic construct
GGKGDDILI

SEQ ID NO: 1012 - protein, 9 aa, synthetic construct
GGSGNDVLK

SEQ ID NO: 1013 - protein, 9 aa, synthetic construct
GGAGADILN

SEQ ID NO: 1014 - protein, 9 aa, synthetic construct
GGEGNDILR

SEQ ID NO: 1015 - protein, 9 aa, synthetic construct
GGAGNDTLG

SEQ ID NO: 1016 - protein, 9 aa, synthetic construct
GGSGDDTLW

SEQ ID NO: 1017 - protein, 9 aa, synthetic construct
GGTGNDTMY

SEQ ID NO: 1018 - protein, 9 aa, synthetic construct
GGAGDDQLD

SEQ ID NO: 1019 - protein, 9 aa, synthetic construct
GGAGDDLIE

SEQ ID NO: 1020 - protein, 9 aa, synthetic construct
GGEGADTFR

SEQ ID NO: 1021 - protein, 9 aa, synthetic construct
GGAGDDVYI

SEQ ID NO: 1022 - protein, 9 aa, synthetic construct
GGAGDDRIT

SEQ ID NO: 1023 - protein, 9 aa, synthetic construct
GGAGDDLLY

SEQ ID NO: 1024 - protein, 9 aa, synthetic construct
GGRGDDWLD

SEQ ID NO: 1025 - protein, 9 aa, synthetic construct
GGDGDDLFK

SEQ ID NO: 1026 - protein, 9 aa, synthetic construct
GGLGKDTLL

SEQ ID NO: 1027 - protein, 9 aa, synthetic construct
GGAGDDLLL

SEQ ID NO: 1028 - protein, 9 aa, synthetic construct
GGVGKDIMT

SEQ ID NO: 1029 - protein, 9 aa, synthetic construct
GGTGADSLY

SEQ ID NO: 1030 - protein, 9 aa, synthetic construct
GGTGDDTLS

SEQ ID NO: 1031 - protein, 9 aa, synthetic construct
GGLGADTLD

SEQ ID NO: 1032 - protein, 9 aa, synthetic construct
GGAGDDSLT

SEQ ID NO: 1033 - protein, 9 aa, synthetic construct
GGGGNDILI

SEQ ID NO: 1034 - protein, 9 aa, synthetic construct
GGTGNDIYV

SEQ ID NO: 1035 - protein, 9 aa, synthetic construct
GGGGNDLLI

SEQ ID NO: 1036 - protein, 9 aa, synthetic construct
GGRGGDRLL

SEQ ID NO: 1037 - protein, 9 aa, synthetic construct
GGAGADILS

SEQ ID NO: 1038 - protein, 9 aa, synthetic construct
GGLGNDTFV

SEQ ID NO: 1039 - protein, 9 aa, synthetic construct
GGGGADLLD

SEQ ID NO: 1040 - protein, 9 aa, synthetic construct
GGLGNDTYF

SEQ ID NO: 1041 - protein, 9 aa, synthetic construct
GGDGDDVLN

SEQ ID NO: 1042 - protein, 9 aa, synthetic construct
GGQGNDTLT

SEQ ID NO: 1043 - protein, 9 aa, synthetic construct
GGTGNDTYY

SEQ ID NO: 1044 - protein, 9 aa, synthetic construct
GGAGTDTLY

SEQ ID NO: 1045 - protein, 9 aa, synthetic construct
GGAGGDLLD

SEQ ID NO: 1046 - protein, 9 aa, synthetic construct
GGEGNDGLA

SEQ ID NO: 1047 - protein, 9 aa, synthetic construct
GGSGNDTYI

SEQ ID NO: 1048 - protein, 9 aa, synthetic construct
GGLGNDLLH

SEQ ID NO: 1049 - protein, 9 aa, synthetic construct
GGSGNDTAS

SEQ ID NO: 1050 - protein, 9 aa, synthetic construct
GGTGNDVLD

SEQ ID NO: 1051 - protein, 9 aa, synthetic construct
GGAGDDVYV

SEQ ID NO: 1052 - protein, 9 aa, synthetic construct
GGAGNDVYV

SEQ ID NO: 1053 - protein, 9 aa, synthetic construct
GGAGADTII

SEQ ID NO: 1054 - protein, 9 aa, synthetic construct
GGAGADTIS

SEQ ID NO: 1055 - protein, 9 aa, synthetic construct
GGKGNDRLI

SEQ ID NO: 1056 - protein, 9 aa, synthetic construct
GGSGNDLLV

SEQ ID NO: 1057 - protein, 9 aa, synthetic construct
GGIGNDILT

SEQ ID NO: 1058 - protein, 9 aa, synthetic construct
GGLGDDLVI

SEQ ID NO: 1059 - protein, 9 aa, synthetic construct
GGAGNDTMI

SEQ ID NO: 1060 - protein, 9 aa, synthetic construct
GGSGADRFV

SEQ ID NO: 1061 - protein, 9 aa, synthetic construct
GGAGADVLS

SEQ ID NO: 1062 - protein, 9 aa, synthetic construct
GGAGRDVFV

SEQ ID NO: 1063 - protein, 9 aa, synthetic construct
GGAGDDTIS

SEQ ID NO: 1064 - protein, 9 aa, synthetic construct
GGTGNDTLM

SEQ ID NO: 1065 - protein, 9 aa, synthetic construct
GGAGNDAVA

SEQ ID NO: 1066 - protein, 9 aa, synthetic construct
GGAGSDTLY

SEQ ID NO: 1067 - protein, 9 aa, synthetic construct
GGSGDDTMT

SEQ ID NO: 1068 - protein, 9 aa, synthetic construct
GGAGSDTLS

SEQ ID NO: 1069 - protein, 9 aa, synthetic construct
GGQGNDTID

SEQ ID NO: 1070 - protein, 9 aa, synthetic construct
GGLGNDVLA

SEQ ID NO: 1071 - protein, 9 aa, synthetic construct
GGAGNDSFV

SEQ ID NO: 1072 - protein, 9 aa, synthetic construct
GGAGNDTMD

SEQ ID NO: 1073 - protein, 9 aa, synthetic construct
GGTGNDILN

SEQ ID NO: 1074 - protein, 9 aa, synthetic construct
GGTGADLMN

SEQ ID NO: 1075 - protein, 9 aa, synthetic construct
GGSGNDLLS

SEQ ID NO: 1076 - protein, 9 aa, synthetic construct
GGAGHDLLH

SEQ ID NO: 1077 - protein, 9 aa, synthetic construct
GGDGNDFLY

SEQ ID NO: 1078 - protein, 9 aa, synthetic construct
GGAGADTFA

SEQ ID NO: 1079 - protein, 9 aa, synthetic construct
GGDGNDRLS

SEQ ID NO: 1080 - protein, 9 aa, synthetic construct
GGKGDDIYI

SEQ ID NO: 1081 - protein, 9 aa, synthetic construct
GGAGDDRLA

SEQ ID NO: 1082 - protein, 9 aa, synthetic construct
GGDGNDTIS

SEQ ID NO: 1083 - protein, 9 aa, synthetic construct
GGGGQDQLS

SEQ ID NO: 1084 - protein, 9 aa, synthetic construct
GGDGDDRLY

SEQ ID NO: 1085 - protein, 9 aa, synthetic construct
GGSGDDTLN

SEQ ID NO: 1086 - protein, 9 aa, synthetic construct
GGAGNDWLS

SEQ ID NO: 1087 - protein, 9 aa, synthetic construct
GGLGNDTIY

SEQ ID NO: 1088 - protein, 9 aa, synthetic construct
GGNGNDSLY

SEQ ID NO: 1089 - protein, 9 aa, synthetic construct
GGTGNDIFV

SEQ ID NO: 1090 - protein, 9 aa, synthetic construct
GGAGNDFLE

SEQ ID NO: 1091 - protein, 9 aa, synthetic construct
GGAGIDIVS

SEQ ID NO: 1092 - protein, 9 aa, synthetic construct
GGDGNDELY

SEQ ID NO: 1093 - protein, 9 aa, synthetic construct
GGNGNDTLT

SEQ ID NO: 1094 - protein, 9 aa, synthetic construct
GGSGDDVLY

SEQ ID NO: 1095 - protein, 9 aa, synthetic construct
GGAGLDTMI

SEQ ID NO: 1096 - protein, 9 aa, synthetic construct
GGGGDDTLN

SEQ ID NO: 1097 - protein, 9 aa, synthetic construct
GGAGNDWLW

SEQ ID NO: 1098 - protein, 9 aa, synthetic construct
GGTGNDLLI

SEQ ID NO: 1099 - protein, 9 aa, synthetic construct
GGLGTDILT

SEQ ID NO: 1100 - protein, 9 aa, synthetic construct
GGDGNDRLI

SEQ ID NO: 1101 - protein, 9 aa, synthetic construct
GGAGNDALF

SEQ ID NO: 1102 - protein, 9 aa, synthetic construct
GGRGDDTLS

SEQ ID NO: 1103 - protein, 9 aa, synthetic construct
GGAGRDNLT

SEQ ID NO: 1104 - protein, 9 aa, synthetic construct
GGAGNDRID

SEQ ID NO: 1105 - protein, 9 aa, synthetic construct
GGAGADTMA

SEQ ID NO: 1106 - protein, 9 aa, synthetic construct
GGAGADILV

SEQ ID NO: 1107 - protein, 9 aa, synthetic construct
GGAGDDNLS

SEQ ID NO: 1108 - protein, 9 aa, synthetic construct
GGAGRDIFL

SEQ ID NO: 1109 - protein, 9 aa, synthetic construct
GGGGADTLV

SEQ ID NO: 1110 - protein, 9 aa, synthetic construct
GGAGDDRLI

SEQ ID NO: 1111 - protein, 9 aa, synthetic construct
GGEGDDTLR

SEQ ID NO: 1112 - protein, 9 aa, synthetic construct
GGAGNDQIF

SEQ ID NO: 1113 - protein, 9 aa, synthetic construct
GGRGNDTLI

SEQ ID NO: 1114 - protein, 9 aa, synthetic construct
GGLGHDRLY

SEQ ID NO: 1115 - protein, 9 aa, synthetic construct
GGTGNDTIT

SEQ ID NO: 1116 - protein, 9 aa, synthetic construct
GGFGHDLLN

SEQ ID NO: 1117 - protein, 9 aa, synthetic construct
GGEGDDSLS

SEQ ID NO: 1118 - protein, 9 aa, synthetic construct
GGTGNDTIN

SEQ ID NO: 1119 - protein, 9 aa, synthetic construct
GGAGTDTLI

SEQ ID NO: 1120 - protein, 9 aa, synthetic construct
GGAGSDVFV

SEQ ID NO: 1121 - protein, 9 aa, synthetic construct
GGGGADSFV

SEQ ID NO: 1122 - protein, 9 aa, synthetic construct
GGAGDDILE

SEQ ID NO: 1123 - protein, 9 aa, synthetic construct
GGDGPDILF

SEQ ID NO: 1124 - protein, 9 aa, synthetic construct
GGSGNDVIV

SEQ ID NO: 1125 - protein, 9 aa, synthetic construct
GGAGDDYLN

SEQ ID NO: 1126 - protein, 9 aa, synthetic construct
GGAGNDTMS

SEQ ID NO: 1127 - protein, 9 aa, synthetic construct
GGTGNDRLY

SEQ ID NO: 1128 - protein, 9 aa, synthetic construct
GGKGDDRIS

SEQ ID NO: 1129 - protein, 9 aa, synthetic construct
GGAGNDFLD

SEQ ID NO: 1130 - protein, 9 aa, synthetic construct
GGGGADILN

SEQ ID NO: 1131 - protein, 9 aa, synthetic construct
GGAGEDTLF

SEQ ID NO: 1132 - protein, 9 aa, synthetic construct
GGIGNDTLY

SEQ ID NO: 1133 - protein, 9 aa, synthetic construct
GGDGDDTLF

SEQ ID NO: 1134 - protein, 9 aa, synthetic construct
GGAGRDTLE

SEQ ID NO: 1135 - protein, 9 aa, synthetic construct
GGTGDDTLL

SEQ ID NO: 1136 - protein, 9 aa, synthetic construct
GGLGSDTLT

SEQ ID NO: 1137 - protein, 9 aa, synthetic construct
GGLGADKLT

SEQ ID NO: 1138 - protein, 9 aa, synthetic construct
GGGGSDTLI

SEQ ID NO: 1139 - protein, 9 aa, synthetic construct
GGAGADLFV

SEQ ID NO: 1140 - protein, 9 aa, synthetic construct
GGSGNDTFV

SEQ ID NO: 1141 - protein, 9 aa, synthetic construct
GGQGDDSLR

SEQ ID NO: 1142 - protein, 9 aa, synthetic construct
GGAGSDTLR

SEQ ID NO: 1143 - protein, 9 aa, synthetic construct
GGYGNDILN

SEQ ID NO: 1144 - protein, 9 aa, synthetic construct
GGTGNDTLH

SEQ ID NO: 1145 - protein, 9 aa, synthetic construct
GGLGNDVLT

SEQ ID NO: 1146 - protein, 9 aa, synthetic construct
GGAGADIFV

SEQ ID NO: 1147 - protein, 9 aa, synthetic construct
GGLGADVLT

SEQ ID NO: 1148 - protein, 9 aa, synthetic construct
GGSGNDVLT

SEQ ID NO: 1149 - protein, 9 aa, synthetic construct
GGLGNDRLI

SEQ ID NO: 1150 - protein, 9 aa, synthetic construct
GGLGNDFID

SEQ ID NO: 1151 - protein, 9 aa, synthetic construct
GGDGDDIIT

SEQ ID NO: 1152 - protein, 9 aa, synthetic construct
GGNGNDILL

SEQ ID NO: 1153 - protein, 9 aa, synthetic construct
GGGGNDTLF

SEQ ID NO: 1154 - protein, 9 aa, synthetic construct
GGSGNDLLF

SEQ ID NO: 1155 - protein, 9 aa, synthetic construct
GGYGKDTIS

SEQ ID NO: 1156 - protein, 9 aa, synthetic construct
GGAGNDILA

SEQ ID NO: 1157 - protein, 9 aa, synthetic construct
GGNGNDRLI

SEQ ID NO: 1158 - protein, 9 aa, synthetic construct
GGAGADTLK

SEQ ID NO: 1159 - protein, 9 aa, synthetic construct
GGLGKDVLT

SEQ ID NO: 1160 - protein, 9 aa, synthetic construct
GGLGKDTLT

SEQ ID NO: 1161 - protein, 9 aa, synthetic construct
GGDGNDLLL

SEQ ID NO: 1162 - protein, 9 aa, synthetic construct
GGTGDDLLI

SEQ ID NO: 1163 - protein, 9 aa, synthetic construct
GGGGNDILR

SEQ ID NO: 1164 - protein, 9 aa, synthetic construct
GGEGNDFLS

SEQ ID NO: 1165 - protein, 9 aa, synthetic construct
GGTGNDTID

SEQ ID NO: 1166 - protein, 9 aa, synthetic construct
GGDGDDVLY

SEQ ID NO: 1167 - protein, 9 aa, synthetic construct
GGLGDDVLI

SEQ ID NO: 1168 - protein, 9 aa, synthetic construct
GGGGNDTFV

SEQ ID NO: 1169 - protein, 9 aa, synthetic construct
GGAGDDILA

SEQ ID NO: 1170 - protein, 9 aa, synthetic construct
GGAGNDKIY

SEQ ID NO: 1171 - protein, 9 aa, synthetic construct
GGTGNDSLS

SEQ ID NO: 1172 - protein, 9 aa, synthetic construct
GGAGNDTFR

SEQ ID NO: 1173 - protein, 9 aa, synthetic construct
GGLGADILI

SEQ ID NO: 1174 - protein, 9 aa, synthetic construct
GGTGNDYLT

SEQ ID NO: 1175 - protein, 9 aa, synthetic construct
GGRGNDTLD

SEQ ID NO: 1176 - protein, 9 aa, synthetic construct
GGDGNDVLM

SEQ ID NO: 1177 - protein, 9 aa, synthetic construct
GGAGADRME

SEQ ID NO: 1178 - protein, 9 aa, synthetic construct
GGAGNDSLA

SEQ ID NO: 1179 - protein, 9 aa, synthetic construct
GGTGNDVLA

SEQ ID NO: 1180 - protein, 9 aa, synthetic construct
GGKGNDVLT

SEQ ID NO: 1181 - protein, 9 aa, synthetic construct
GGGGADTLS

SEQ ID NO: 1182 - protein, 9 aa, synthetic construct
GGNGDDLLI

SEQ ID NO: 1183 - protein, 9 aa, synthetic construct
GGAGNDTIE

SEQ ID NO: 1184 - protein, 9 aa, synthetic construct
GGAGVDVLK

SEQ ID NO: 1185 - protein, 9 aa, synthetic construct
GGSGADTLN

SEQ ID NO: 1186 - protein, 9 aa, synthetic construct
GGIGNDTLS

SEQ ID NO: 1187 - protein, 9 aa, synthetic construct
GGAGDDLLR

SEQ ID NO: 1188 - protein, 9 aa, synthetic construct
GGQGNDILT

SEQ ID NO: 1189 - protein, 9 aa, synthetic construct
GGAGADTMV

SEQ ID NO: 1190 - protein, 9 aa, synthetic construct
GGGGVDYAW

SEQ ID NO: 1191 - protein, 9 aa, synthetic construct
GGAGADYMD

SEQ ID NO: 1192 - protein, 9 aa, synthetic construct
GGAGNDKLN

SEQ ID NO: 1193 - protein, 9 aa, synthetic construct
GGDGHDKLY

SEQ ID NO: 1194 - protein, 9 aa, synthetic construct
GGAGADQLV

SEQ ID NO: 1195 - protein, 9 aa, synthetic construct
GGSGNDSLS

SEQ ID NO: 1196 - protein, 9 aa, synthetic construct
GGQGNDQLS

SEQ ID NO: 1197 - protein, 9 aa, synthetic construct
GGAGADLLS

SEQ ID NO: 1198 - protein, 9 aa, synthetic construct
GGAGQDVLI

SEQ ID NO: 1199 - protein, 9 aa, synthetic construct
GGAGDDVIR

SEQ ID NO: 1200 - protein, 9 aa, synthetic construct
GGTGNDTIY

SEQ ID NO: 1201 - protein, 9 aa, synthetic construct
GGAGNDNLN

SEQ ID NO: 1202 - protein, 9 aa, synthetic construct
GGKGNDILV

SEQ ID NO: 1203 - protein, 9 aa, synthetic construct
GGSGNDVLV

SEQ ID NO: 1204 - protein, 9 aa, synthetic construct
GGAGDDTLK

SEQ ID NO: 1205 - protein, 9 aa, synthetic construct
GGAGADVMI

SEQ ID NO: 1206 - protein, 9 aa, synthetic construct
GGAGNDQLI

SEQ ID NO: 1207 - protein, 9 aa, synthetic construct
GGSGDDLLD

SEQ ID NO: 1208 - protein, 9 aa, synthetic construct
GGAGDDTYF

SEQ ID NO: 1209 - protein, 9 aa, synthetic construct
GGAGADIMI

SEQ ID NO: 1210 - protein, 9 aa, synthetic construct
GGDGNDHLY

SEQ ID NO: 1211 - protein, 9 aa, synthetic construct
GGAGSDTAS

SEQ ID NO: 1212 - protein, 9 aa, synthetic construct
GGAGSDILI

SEQ ID NO: 1213 - protein, 9 aa, synthetic construct
GGQGDDTLT

SEQ ID NO: 1214 - protein, 9 aa, synthetic construct
GGSGDDTLT

SEQ ID NO: 1215 - protein, 9 aa, synthetic construct
GGDGSDTLT

SEQ ID NO: 1216 - protein, 9 aa, synthetic construct
GGEGDDTFV

SEQ ID NO: 1217 - protein, 9 aa, synthetic construct
GGEGADVFV

SEQ ID NO: 1218 - protein, 9 aa, synthetic construct
GGAGDDRLL

SEQ ID NO: 1219 - protein, 9 aa, synthetic construct
GGAGDDSID

SEQ ID NO: 1220 - protein, 9 aa, synthetic construct
GGAGTDTLS

SEQ ID NO: 1221 - protein, 9 aa, synthetic construct
GGAGADSLV

SEQ ID NO: 1222 - protein, 9 aa, synthetic construct
GGKGDDLLF

SEQ ID NO: 1223 - protein, 9 aa, synthetic construct
GGAGNDTIR

SEQ ID NO: 1224 - protein, 9 aa, synthetic construct
GGGGDDTLS

SEQ ID NO: 1225 - protein, 9 aa, synthetic construct
GGTGVDTLI

SEQ ID NO: 1226 - protein, 9 aa, synthetic construct
GGDGNDTVD

SEQ ID NO: 1227 - protein, 9 aa, synthetic construct
GGAGNDILE

SEQ ID NO: 1228 - protein, 9 aa, synthetic construct
GGVGHDYMD

SEQ ID NO: 1229 - protein, 9 aa, synthetic construct
GGAGADTMD

SEQ ID NO: 1230 - protein, 9 aa, synthetic construct
GGTGNDVLV

SEQ ID NO: 1231 - protein, 9 aa, synthetic construct
GGTGDDVLT

SEQ ID NO: 1232 - protein, 9 aa, synthetic construct
GGAGDDALS

SEQ ID NO: 1233 - protein, 9 aa, synthetic construct
GGEGDDDLY

SEQ ID NO: 1234 - protein, 9 aa, synthetic construct
GGEGNDTLF

SEQ ID NO: 1235 - protein, 9 aa, synthetic construct
GGDGNDYLV

SEQ ID NO: 1236 - protein, 9 aa, synthetic construct
GGVGNDTIW

SEQ ID NO: 1237 - protein, 9 aa, synthetic construct
GGAGHDTLN

SEQ ID NO: 1238 - protein, 9 aa, synthetic construct
GGEGNDTLK

SEQ ID NO: 1239 - protein, 9 aa, synthetic construct
GGDGDDIID

SEQ ID NO: 1240 - protein, 9 aa, synthetic construct
GGDGDDSLL

SEQ ID NO: 1241 - protein, 9 aa, synthetic construct
GGDGADTLR

SEQ ID NO: 1242 - protein, 9 aa, synthetic construct
GGDGADVLR

SEQ ID NO: 1243 - protein, 9 aa, synthetic construct
GGQGNDTLD

SEQ ID NO: 1244 - protein, 9 aa, synthetic construct
GGDGDDVLS

SEQ ID NO: 1245 - protein, 9 aa, synthetic construct
GGAGNDILQ

SEQ ID NO: 1246 - protein, 9 aa, synthetic construct
GGGGADQFI

SEQ ID NO: 1247 - protein, 9 aa, synthetic construct
GGDGNDTYY

SEQ ID NO: 1248 - protein, 9 aa, synthetic construct
GGLGGDHLW

SEQ ID NO: 1249 - protein, 9 aa, synthetic construct
GGSGADEVR

SEQ ID NO: 1250 - protein, 9 aa, synthetic construct
GGGGADRLE

SEQ ID NO: 1251 - protein, 9 aa, synthetic construct
GGAGNDIFV

SEQ ID NO: 1252 - protein, 9 aa, synthetic construct
GGGGNDTLK

SEQ ID NO: 1253 - protein, 9 aa, synthetic construct
GGAGDDLLQ

SEQ ID NO: 1254 - protein, 9 aa, synthetic construct
GGDGNDNLQ

SEQ ID NO: 1255 - protein, 9 aa, synthetic construct
GGDGDDKLY

SEQ ID NO: 1256 - protein, 9 aa, synthetic construct
GGAGDDRIL

SEQ ID NO: 1257 - protein, 9 aa, synthetic construct
GGYGNDTLS

SEQ ID NO: 1258 - protein, 9 aa, synthetic construct
GGEGDDQLS

SEQ ID NO: 1259 - protein, 9 aa, synthetic construct
GGLGADTLV

SEQ ID NO: 1260 - protein, 9 aa, synthetic construct
GGAGDDLLT

SEQ ID NO: 1261 - protein, 9 aa, synthetic construct
GGTGNDSLT

SEQ ID NO: 1262 - protein, 9 aa, synthetic construct
GGAGDDSLL

SEQ ID NO: 1263 - protein, 9 aa, synthetic construct
GGAGNDTIH

SEQ ID NO: 1264 - protein, 9 aa, synthetic construct
GGAGNDTVS

SEQ ID NO: 1265 - protein, 9 aa, synthetic construct
GGAGDDSLN

SEQ ID NO: 1266 - protein, 9 aa, synthetic construct
GGEGDDTIL

SEQ ID NO: 1267 - protein, 9 aa, synthetic construct
GGAGNDSIN

SEQ ID NO: 1268 - protein, 9 aa, synthetic construct
GGAGKDTFI

SEQ ID NO: 1269 - protein, 9 aa, synthetic construct
GGLGNDTIN

SEQ ID NO: 1270 - protein, 9 aa, synthetic construct
GGTGADTLV

SEQ ID NO: 1271 - protein, 9 aa, synthetic construct
GGKGDDTLA

SEQ ID NO: 1272 - protein, 9 aa, synthetic construct
GGAGKDVFV

SEQ ID NO: 1273 - protein, 9 aa, synthetic construct
GGGGDDRLD

SEQ ID NO: 1274 - protein, 9 aa, synthetic construct
GGAGNDHLF

SEQ ID NO: 1275 - protein, 9 aa, synthetic construct
GGDGDDQLF

SEQ ID NO: 1276 - protein, 9 aa, synthetic construct
GGDGDDRLV

SEQ ID NO: 1277 - protein, 9 aa, synthetic construct
GGEGTDTLA

SEQ ID NO: 1278 - protein, 9 aa, synthetic construct
GGGGADQFF

SEQ ID NO: 1279 - protein, 9 aa, synthetic construct
GGLGDDLLN

SEQ ID NO: 1280 - protein, 9 aa, synthetic construct
GGEGNDYLD

SEQ ID NO: 1281 - protein, 9 aa, synthetic construct
GGKGDDVII

SEQ ID NO: 1282 - protein, 9 aa, synthetic construct
GGKGNDYLE

SEQ ID NO: 1283 - protein, 9 aa, synthetic construct
GGPGNDTLA

SEQ ID NO: 1284 - protein, 9 aa, synthetic construct
GGTGNDELH

SEQ ID NO: 1285 - protein, 9 aa, synthetic construct
GGGGDDTLT

SEQ ID NO: 1286 - protein, 9 aa, synthetic construct
GGGGSDYIL

SEQ ID NO: 1287 - protein, 9 aa, synthetic construct
GGKGNDVIN

SEQ ID NO: 1288 - protein, 9 aa, synthetic construct
GGAGGDTLD

SEQ ID NO: 1289 - protein, 9 aa, synthetic construct
GGSGNDIYL

SEQ ID NO: 1290 - protein, 9 aa, synthetic construct
GGAGNDTFI

SEQ ID NO: 1291 - protein, 9 aa, synthetic construct
GGAGDDWLT

SEQ ID NO: 1292 - protein, 9 aa, synthetic construct
GGAGADVFA

SEQ ID NO: 1293 - protein, 9 aa, synthetic construct
GGDGDDILN

SEQ ID NO: 1294 - protein, 9 aa, synthetic construct
GGSGNDHIY

SEQ ID NO: 1295 - protein, 9 aa, synthetic construct
GGYGDDIYR

SEQ ID NO: 1296 - protein, 9 aa, synthetic construct
GGVGADTLI

SEQ ID NO: 1297 - protein, 9 aa, synthetic construct
GGVGNDTLS

SEQ ID NO: 1298 - protein, 9 aa, synthetic construct
GGEGDDTLD

SEQ ID NO: 1299 - protein, 9 aa, synthetic construct
GGGGADTFL

SEQ ID NO: 1300 - protein, 9 aa, synthetic construct
GGAGDDYLS

SEQ ID NO: 1301 - protein, 9 aa, synthetic construct
GGDGNDILF

SEQ ID NO: 1302 - protein, 9 aa, synthetic construct
GGQGNDTYV

SEQ ID NO: 1303 - protein, 9 aa, synthetic construct
GGEGVDQLS

SEQ ID NO: 1304 - protein, 9 aa, synthetic construct
GGDGADTID

SEQ ID NO: 1305 - protein, 9 aa, synthetic construct
GGDGNDVYI

SEQ ID NO: 1306 - protein, 9 aa, synthetic construct
GGDGDDTLM

SEQ ID NO: 1307 - protein, 9 aa, synthetic construct
GGEGADTLS

SEQ ID NO: 1308 - protein, 9 aa, synthetic construct
GGKGNDTLD

SEQ ID NO: 1309 - protein, 9 aa, synthetic construct
GGAGADRLR

SEQ ID NO: 1310 - protein, 9 aa, synthetic construct
GGTGNDLLV

SEQ ID NO: 1311 - protein, 9 aa, synthetic construct
GGAGNDLLA

SEQ ID NO: 1312 - protein, 9 aa, synthetic construct
GGAGDDTIT

SEQ ID NO: 1313 - protein, 9 aa, synthetic construct
GGAGNDIID

SEQ ID NO: 1314 - protein, 9 aa, synthetic construct
GGAGNDLIE

SEQ ID NO: 1315 - protein, 9 aa, synthetic construct
GGAGDDILL

SEQ ID NO: 1316 - protein, 9 aa, synthetic construct
GGKGMDTLK

SEQ ID NO: 1317 - protein, 9 aa, synthetic construct
GGLGSDLLD

SEQ ID NO: 1318 - protein, 9 aa, synthetic construct
GGTGDDVLR

SEQ ID NO: 1319 - protein, 9 aa, synthetic construct
GGAGNDKLE

SEQ ID NO: 1320 - protein, 9 aa, synthetic construct
GGVGNDTLF

SEQ ID NO: 1321 - protein, 9 aa, synthetic construct
GGEGADNLQ

SEQ ID NO: 1322 - protein, 9 aa, synthetic construct
GGSGADTLA

SEQ ID NO: 1323 - protein, 9 aa, synthetic construct
GGTGNDTYN

SEQ ID NO: 1324 - protein, 9 aa, synthetic construct
GGSGADTFL

SEQ ID NO: 1325 - protein, 9 aa, synthetic construct
GGTGNDRLD

SEQ ID NO: 1326 - protein, 9 aa, synthetic construct
GGAGDDSLV

SEQ ID NO: 1327 - protein, 9 aa, synthetic construct
GGVGNDLLD

SEQ ID NO: 1328 - protein, 9 aa, synthetic construct
GGAGDDFLS

SEQ ID NO: 1329 - protein, 9 aa, synthetic construct
GGVGNDTYV

SEQ ID NO: 1330 - protein, 9 aa, synthetic construct
GGGGADTLN

SEQ ID NO: 1331 - protein, 9 aa, synthetic construct
GGFGHDRVN

SEQ ID NO: 1332 - protein, 9 aa, synthetic construct
GGNGIDTAD

SEQ ID NO: 1333 - protein, 9 aa, synthetic construct
GGAGNDELS

SEQ ID NO: 1334 - protein, 9 aa, synthetic construct
GGSGNDVLR

SEQ ID NO: 1335 - protein, 9 aa, synthetic construct
GGQGNDVLT

SEQ ID NO: 1336 - protein, 9 aa, synthetic construct
GGDGNDTLH

SEQ ID NO: 1337 - protein, 9 aa, synthetic construct
GGKGNDTLV

SEQ ID NO: 1338 - protein, 9 aa, synthetic construct
GGDGNDVID

SEQ ID NO: 1339 - protein, 9 aa, synthetic construct
GGLGADSMA

SEQ ID NO: 1340 - protein, 9 aa, synthetic construct
GGAGIDTLN

SEQ ID NO: 1341 - protein, 9 aa, synthetic construct
GGTGNDLLS

SEQ ID NO: 1342 - protein, 9 aa, synthetic construct
GGEGDDTLF

SEQ ID NO: 1343 - protein, 9 aa, synthetic construct
GGAGADHLD

SEQ ID NO: 1344 - protein, 9 aa, synthetic construct
GGSGADTLS

SEQ ID NO: 1345 - protein, 9 aa, synthetic construct
GGGGDDTLD

SEQ ID NO: 1346 - protein, 9 aa, synthetic construct
GGDGDDIFK

SEQ ID NO: 1347 - protein, 9 aa, synthetic construct
GGEGNDVLI

SEQ ID NO: 1348 - protein, 9 aa, synthetic construct
GGNGDDTYD

SEQ ID NO: 1349 - protein, 9 aa, synthetic construct
GGGGNDVLT

SEQ ID NO: 1350 - protein, 9 aa, synthetic construct
GGTGRDTID

SEQ ID NO: 1351 - protein, 9 aa, synthetic construct
GGAGADTAI

SEQ ID NO: 1352 - protein, 9 aa, synthetic construct
GGSGDDRIE

SEQ ID NO: 1353 - protein, 9 aa, synthetic construct
GGAGVDTVD

SEQ ID NO: 1354 - protein, 9 aa, synthetic construct
GGSGADTLL

SEQ ID NO: 1355 - protein, 9 aa, synthetic construct
GGDGDDVLH

SEQ ID NO: 1356 - protein, 9 aa, synthetic construct
GGAGTDTLN

SEQ ID NO: 1357 - protein, 9 aa, synthetic construct
GGLGADRLT

SEQ ID NO: 1358 - protein, 9 aa, synthetic construct
GGAGNDFLI

SEQ ID NO: 1359 - protein, 9 aa, synthetic construct
GGHGDDTLI

SEQ ID NO: 1360 - protein, 9 aa, synthetic construct
GGNGDDVLL

SEQ ID NO: 1361 - protein, 9 aa, synthetic construct
GGTGNDTMR

SEQ ID NO: 1362 - protein, 9 aa, synthetic construct
GGSGDDTLR

SEQ ID NO: 1363 - protein, 9 aa, synthetic construct
GGAGADQFV

SEQ ID NO: 1364 - protein, 9 aa, synthetic construct
GGGGSDTLV

SEQ ID NO: 1365 - protein, 9 aa, synthetic construct
GGGGNDSLD

SEQ ID NO: 1366 - protein, 9 aa, synthetic construct
GGAGADRFI

SEQ ID NO: 1367 - protein, 9 aa, synthetic construct
GGAGDDYLY

SEQ ID NO: 1368 - protein, 9 aa, synthetic construct
GGGGADTLA

SEQ ID NO: 1369 - protein, 9 aa, synthetic construct
GGAGDDLIL

SEQ ID NO: 1370 - protein, 9 aa, synthetic construct
GGAGDDDLT

SEQ ID NO: 1371 - protein, 9 aa, synthetic construct
GGAGADSLL

SEQ ID NO: 1372 - protein, 9 aa, synthetic construct
GGIGNDTLR

SEQ ID NO: 1373 - protein, 9 aa, synthetic construct
GGRGADTFV

SEQ ID NO: 1374 - protein, 9 aa, synthetic construct
GGEGDDTID

SEQ ID NO: 1375 - protein, 9 aa, synthetic construct
GGSGDDTLV

SEQ ID NO: 1376 - protein, 9 aa, synthetic construct
GGTGADTID

SEQ ID NO: 1377 - protein, 9 aa, synthetic construct
GGTGNDILY

SEQ ID NO: 1378 - protein, 9 aa, synthetic construct
GGDGNDHIY

SEQ ID NO: 1379 - protein, 9 aa, synthetic construct
GGAGNDHLD

SEQ ID NO: 1380 - protein, 9 aa, synthetic construct
GGTGNDKMT

SEQ ID NO: 1381 - protein, 9 aa, synthetic construct
GGSGNDTLH

SEQ ID NO: 1382 - protein, 9 aa, synthetic construct
GGNGNDTLR

SEQ ID NO: 1383 - protein, 9 aa, synthetic construct
GGRGEDTLI

SEQ ID NO: 1384 - protein, 9 aa, synthetic construct
GGTGADRMT

SEQ ID NO: 1385 - protein, 9 aa, synthetic construct
GGDGFDEVT

SEQ ID NO: 1386 - protein, 9 aa, synthetic construct
GGSGNDTIS

SEQ ID NO: 1387 - protein, 9 aa, synthetic construct
GGAGIDTLT

SEQ ID NO: 1388 - protein, 9 aa, synthetic construct
GGTGNDRLF

SEQ ID NO: 1389 - protein, 9 aa, synthetic construct
GGAGNDTIA

SEQ ID NO: 1390 - protein, 9 aa, synthetic construct
GGPGNDLLD

SEQ ID NO: 1391 - protein, 9 aa, synthetic construct
GGAGRDLIY

SEQ ID NO: 1392 - protein, 9 aa, synthetic construct
GGVGSDTLS

SEQ ID NO: 1393 - protein, 9 aa, synthetic construct
GGEGNDVLK

SEQ ID NO: 1394 - protein, 9 aa, synthetic construct
GGEGNDVLD

SEQ ID NO: 1395 - protein, 9 aa, synthetic construct
GGEGRDVMY

SEQ ID NO: 1396 - protein, 9 aa, synthetic construct
GGGGNDTIN

SEQ ID NO: 1397 - protein, 9 aa, synthetic construct
GGAGADTML

SEQ ID NO: 1398 - protein, 9 aa, synthetic construct
GGQGDDLLD

SEQ ID NO: 1399 - protein, 9 aa, synthetic construct
GGGGDDIFK

SEQ ID NO: 1400 - protein, 9 aa, synthetic construct
GGAGADRMR

SEQ ID NO: 1401 - protein, 9 aa, synthetic construct
GGSGADILF

SEQ ID NO: 1402 - protein, 9 aa, synthetic construct
GGLGNDTLV

SEQ ID NO: 1403 - protein, 9 aa, synthetic construct
GGDGNDKLY

SEQ ID NO: 1404 - protein, 9 aa, synthetic construct
GGAGDDVIS

SEQ ID NO: 1405 - protein, 9 aa, synthetic construct
GGNGNDRLD

SEQ ID NO: 1406 - protein, 9 aa, synthetic construct
GGLGDDVLS

SEQ ID NO: 1407 - protein, 9 aa, synthetic construct
GGQGDDIMT

SEQ ID NO: 1408 - protein, 9 aa, synthetic construct
GGAGNDVMH

SEQ ID NO: 1409 - protein, 9 aa, synthetic construct
GGEGNDQLF

SEQ ID NO: 1410 - protein, 9 aa, synthetic construct
GGDGADHFV

SEQ ID NO: 1411 - protein, 9 aa, synthetic construct
GGTGIDKMS

SEQ ID NO: 1412 - protein, 9 aa, synthetic construct
GGIGVDTFK

SEQ ID NO: 1413 - protein, 9 aa, synthetic construct
GGAGSDTLF

SEQ ID NO: 1414 - protein, 9 aa, synthetic construct
GGLGSDYLQ

SEQ ID NO: 1415 - protein, 9 aa, synthetic construct
GGTGADLLI

SEQ ID NO: 1416 - protein, 9 aa, synthetic construct
GGAGNDVFR

SEQ ID NO: 1417 - protein, 9 aa, synthetic construct
GGAGADLMI

SEQ ID NO: 1418 - protein, 9 aa, synthetic construct
GGDGDDTIY

SEQ ID NO: 1419 - protein, 9 aa, synthetic construct
GGAGDDQVI

SEQ ID NO: 1420 - protein, 9 aa, synthetic construct
GGAGDDSLY

SEQ ID NO: 1421 - protein, 9 aa, synthetic construct
GGLGDDILS

SEQ ID NO: 1422 - protein, 9 aa, synthetic construct
GGTGNDRLE

SEQ ID NO: 1423 - protein, 9 aa, synthetic construct
GGSGDDTLY

SEQ ID NO: 1424 - protein, 9 aa, synthetic construct
GGAGRDVLY

SEQ ID NO: 1425 - protein, 9 aa, synthetic construct
GGAGNDFLA

SEQ ID NO: 1426 - protein, 9 aa, synthetic construct
GGSGADLFR

SEQ ID NO: 1427 - protein, 9 aa, synthetic construct
GGTGADRLY

SEQ ID NO: 1428 - protein, 9 aa, synthetic construct
GGSGADLFV

SEQ ID NO: 1429 - protein, 9 aa, synthetic construct
GGSGNDELY

SEQ ID NO: 1430 - protein, 9 aa, synthetic construct
GGEGNDTYV

SEQ ID NO: 1431 - protein, 9 aa, synthetic construct
GGSGNDILS

SEQ ID NO: 1432 - protein, 9 aa, synthetic construct
GGAGVDTLV

SEQ ID NO: 1433 - protein, 9 aa, synthetic construct
GGSGNDLLL

SEQ ID NO: 1434 - protein, 9 aa, synthetic construct
GGDGDDTIS

SEQ ID NO: 1435 - protein, 9 aa, synthetic construct
GGDGADTLY

SEQ ID NO: 1436 - protein, 9 aa, synthetic construct
GGTGSDTMT

SEQ ID NO: 1437 - protein, 9 aa, synthetic construct
GGAGDDSLI

SEQ ID NO: 1438 - protein, 9 aa, synthetic construct
GGLGSDVLD

SEQ ID NO: 1439 - protein, 9 aa, synthetic construct
GGDGNDTLK

SEQ ID NO: 1440 - protein, 9 aa, synthetic construct
GGEGDDLLD

SEQ ID NO: 1441 - protein, 9 aa, synthetic construct
GGDGIDTAD

SEQ ID NO: 1442 - protein, 9 aa, synthetic construct
GGDGDDQLT

SEQ ID NO: 1443 - protein, 9 aa, synthetic construct
GGNGDDHLY

SEQ ID NO: 1444 - protein, 9 aa, synthetic construct
GGEGDDTLE

SEQ ID NO: 1445 - protein, 9 aa, synthetic construct
GGLGNDIYI

SEQ ID NO: 1446 - protein, 9 aa, synthetic construct
GGGGNDVLR

SEQ ID NO: 1447 - protein, 9 aa, synthetic construct
GGAGDDLLA

SEQ ID NO: 1448 - protein, 9 aa, synthetic construct
GGFGADTLY

SEQ ID NO: 1449 - protein, 9 aa, synthetic construct
GGLGNDLIN

SEQ ID NO: 1450 - protein, 9 aa, synthetic construct
GGLGNDMLN

SEQ ID NO: 1451 - protein, 9 aa, synthetic construct
GGNGIDILN

SEQ ID NO: 1452 - protein, 9 aa, synthetic construct
GGAGNDVYI

SEQ ID NO: 1453 - protein, 9 aa, synthetic construct
GGSGNDVLS

SEQ ID NO: 1454 - protein, 9 aa, synthetic construct
GGDGDDVLV

SEQ ID NO: 1455 - protein, 9 aa, synthetic construct
GGSGVDTVV

SEQ ID NO: 1456 - protein, 9 aa, synthetic construct
GGDGDDILR

SEQ ID NO: 1457 - protein, 9 aa, synthetic construct
GGRGADSLT

SEQ ID NO: 1458 - protein, 9 aa, synthetic construct
GGGGSDIIK

SEQ ID NO: 1459 - protein, 9 aa, synthetic construct
GGGGADIFV

SEQ ID NO: 1460 - protein, 9 aa, synthetic construct
GGEGSDRYE

SEQ ID NO: 1461 - protein, 9 aa, synthetic construct
GGLGADVMV

SEQ ID NO: 1462 - protein, 9 aa, synthetic construct
GGIGNDTLT

SEQ ID NO: 1463 - protein, 9 aa, synthetic construct
GGEGDDTLY

SEQ ID NO: 1464 - protein, 9 aa, synthetic construct
GGLGADTFE

SEQ ID NO: 1465 - protein, 9 aa, synthetic construct
GGLGDDQLY

SEQ ID NO: 1466 - protein, 9 aa, synthetic construct
GGEGDDSID

SEQ ID NO: 1467 - protein, 9 aa, synthetic construct
GGDGVDTYY

SEQ ID NO: 1468 - protein, 9 aa, synthetic construct
GGAGADSLF

SEQ ID NO: 1469 - protein, 9 aa, synthetic construct
GGDGDDLLR

SEQ ID NO: 1470 - protein, 9 aa, synthetic construct
GGSGADRLD

SEQ ID NO: 1471 - protein, 9 aa, synthetic construct
GGAGADIFR

SEQ ID NO: 1472 - protein, 9 aa, synthetic construct
GGAGDDSLR

SEQ ID NO: 1473 - protein, 9 aa, synthetic construct
GGDGCDTLI

SEQ ID NO: 1474 - protein, 9 aa, synthetic construct
GGLGDDVLT

SEQ ID NO: 1475 - protein, 9 aa, synthetic construct
GGKGADTFV

SEQ ID NO: 1476 - protein, 9 aa, synthetic construct
GGGGDDVLD

SEQ ID NO: 1477 - protein, 9 aa, synthetic construct
GGSGNDSLV

SEQ ID NO: 1478 - protein, 9 aa, synthetic construct
GGSGNDSLF

SEQ ID NO: 1479 - protein, 9 aa, synthetic construct
GGGGSDTFV

SEQ ID NO: 1480 - protein, 9 aa, synthetic construct
GGAGNDFID

SEQ ID NO: 1481 - protein, 9 aa, synthetic construct
GGTGDDTID

SEQ ID NO: 1482 - protein, 9 aa, synthetic construct
GGAGNDDLY

SEQ ID NO: 1483 - protein, 9 aa, synthetic construct
GGSGDDKLY

SEQ ID NO: 1484 - protein, 9 aa, synthetic construct
GGTGADRME

SEQ ID NO: 1485 - protein, 9 aa, synthetic construct
GGAGNDSIV

SEQ ID NO: 1486 - protein, 9 aa, synthetic construct
GGAGDDIYY

SEQ ID NO: 1487 - protein, 9 aa, synthetic construct
GGDGDDVLR

SEQ ID NO: 1488 - protein, 9 aa, synthetic construct
GGAGNDFFV

SEQ ID NO: 1489 - protein, 9 aa, synthetic construct
GGKGNDTYF

SEQ ID NO: 1490 - protein, 9 aa, synthetic construct
GGVGNDILN

SEQ ID NO: 1491 - protein, 9 aa, synthetic construct
GGAGRDTLL

SEQ ID NO: 1492 - protein, 9 aa, synthetic construct
GGLGNDIYV

SEQ ID NO: 1493 - protein, 9 aa, synthetic construct
GGSGDDEMF

SEQ ID NO: 1494 - protein, 9 aa, synthetic construct
GGDGDDFLA

SEQ ID NO: 1495 - protein, 9 aa, synthetic construct
GGKGNDTLY

SEQ ID NO: 1496 - protein, 9 aa, synthetic construct
GGAGGDRLR

SEQ ID NO: 1497 - protein, 9 aa, synthetic construct
GGSGADKLI

SEQ ID NO: 1498 - protein, 9 aa, synthetic construct
GGSGNDRLS

SEQ ID NO: 1499 - protein, 9 aa, synthetic construct
GGDGDDSLS

SEQ ID NO: 1500 - protein, 9 aa, synthetic construct
GGLGNDTYL

SEQ ID NO: 1501 - protein, 9 aa, synthetic construct
GGSGSDTLS

SEQ ID NO: 1502 - protein, 9 aa, synthetic construct
GGAGNDNLT

SEQ ID NO: 1503 - protein, 9 aa, synthetic construct
GGFGYDRVN

SEQ ID NO: 1504 - protein, 9 aa, synthetic construct
GGTGADTLL

SEQ ID NO: 1505 - protein, 9 aa, synthetic construct
GGGGSDTFK

SEQ ID NO: 1506 - protein, 9 aa, synthetic construct
GGAGDDTIL

SEQ ID NO: 1507 - protein, 9 aa, synthetic construct
GGDGDDSLI

SEQ ID NO: 1508 - protein, 9 aa, synthetic construct
GGEGADDFV

SEQ ID NO: 1509 - protein, 9 aa, synthetic construct
GGTGNDQLD

SEQ ID NO: 1510 - protein, 9 aa, synthetic construct
GGVGNDILD

SEQ ID NO: 1511 - protein, 9 aa, synthetic construct
GGVGKDTLI

SEQ ID NO: 1512 - protein, 9 aa, synthetic construct
GGFGFDRVN

SEQ ID NO: 1513 - protein, 9 aa, synthetic construct
GGAGNDIYI

SEQ ID NO: 1514 - protein, 9 aa, synthetic construct
GGNGADTLD

SEQ ID NO: 1515 - protein, 9 aa, synthetic construct
GGEGRDVLY

SEQ ID NO: 1516 - protein, 9 aa, synthetic construct
GGGGADSLW

SEQ ID NO: 1517 - protein, 9 aa, synthetic construct
GGYGDDTLD

SEQ ID NO: 1518 - protein, 9 aa, synthetic construct
GGAGNDIIN

SEQ ID NO: 1519 - protein, 9 aa, synthetic construct
GGAGADVID

SEQ ID NO: 1520 - protein, 9 aa, synthetic construct
GGSGADTMS

SEQ ID NO: 1521 - protein, 9 aa, synthetic construct
GGLGRDTLA

SEQ ID NO: 1522 - protein, 9 aa, synthetic construct
GGNGNDLLL

SEQ ID NO: 1523 - protein, 9 aa, synthetic construct
GGTGNDLLY

SEQ ID NO: 1524 - protein, 9 aa, synthetic construct
GGAGKDVLT

SEQ ID NO: 1525 - protein, 9 aa, synthetic construct
GGAGADTIN

SEQ ID NO: 1526 - protein, 9 aa, synthetic construct
GGAGDDWLE

SEQ ID NO: 1527 - protein, 9 aa, synthetic construct
GGVGDDVIY

SEQ ID NO: 1528 - protein, 9 aa, synthetic construct
GGDGDDLLE

SEQ ID NO: 1529 - protein, 9 aa, synthetic construct
GGAGNDTIQ

SEQ ID NO: 1530 - protein, 9 aa, synthetic construct
GGAGDDALF

SEQ ID NO: 1531 - protein, 9 aa, synthetic construct
GGDGNDQLF

SEQ ID NO: 1532 - protein, 9 aa, synthetic construct
GGGGDDSLS

SEQ ID NO: 1533 - protein, 9 aa, synthetic construct
GGAGNDNIK

SEQ ID NO: 1534 - protein, 9 aa, synthetic construct
GGDGSDVYR

SEQ ID NO: 1535 - protein, 9 aa, synthetic construct
GGGGNDTIF

SEQ ID NO: 1536 - protein, 9 aa, synthetic construct
GGKGHDTLA

SEQ ID NO: 1537 - protein, 9 aa, synthetic construct
GGSGNDRLT

SEQ ID NO: 1538 - protein, 9 aa, synthetic construct
GGDGADTLV

SEQ ID NO: 1539 - protein, 9 aa, synthetic construct
GGAGSDTLL

SEQ ID NO: 1540 - protein, 9 aa, synthetic construct
GGDGDDVLL

SEQ ID NO: 1541 - protein, 9 aa, synthetic construct
GGEGNDIYV

SEQ ID NO: 1542 - protein, 9 aa, synthetic construct
GGGGNDTIS

SEQ ID NO: 1543 - protein, 9 aa, synthetic construct
GGAGKDTLD

SEQ ID NO: 1544 - protein, 9 aa, synthetic construct
GGSGSDRLY

SEQ ID NO: 1545 - protein, 9 aa, synthetic construct
GGSGADSMS

SEQ ID NO: 1546 - protein, 9 aa, synthetic construct
GGVGDDRLV

SEQ ID NO: 1547 - protein, 9 aa, synthetic construct
GGSGKDTFV

SEQ ID NO: 1548 - protein, 9 aa, synthetic construct
GGAGRDVLT

SEQ ID NO: 1549 - protein, 9 aa, synthetic construct
GGSGSDTFV

SEQ ID NO: 1550 - protein, 9 aa, synthetic construct
GGLGNDRLT

SEQ ID NO: 1551 - protein, 9 aa, synthetic construct
GGEGSDTVF

SEQ ID NO: 1552 - protein, 9 aa, synthetic construct
GGAGADVLA

SEQ ID NO: 1553 - protein, 9 aa, synthetic construct
GGAGNDTFN

SEQ ID NO: 1554 - protein, 9 aa, synthetic construct
GGTGTDRLE

SEQ ID NO: 1555 - protein, 9 aa, synthetic construct
GGGGDDVLY

SEQ ID NO: 1556 - protein, 9 aa, synthetic construct
GGDGNDLLE

SEQ ID NO: 1557 - protein, 9 aa, synthetic construct
GGDGNDILQ

SEQ ID NO: 1558 - protein, 9 aa, synthetic construct
GGAGDDRIM

SEQ ID NO: 1559 - protein, 9 aa, synthetic construct
GGSGTDRLD

SEQ ID NO: 1560 - protein, 9 aa, synthetic construct
GGAGNDVIS

SEQ ID NO: 1561 - protein, 9 aa, synthetic construct
GGAGADLLA

SEQ ID NO: 1562 - protein, 9 aa, synthetic construct
GGGGNDTLA

SEQ ID NO: 1563 - protein, 9 aa, synthetic construct
GGLGDDVLD

SEQ ID NO: 1564 - protein, 9 aa, synthetic construct
GGDGDDVIE

SEQ ID NO: 1565 - protein, 9 aa, synthetic construct
GGAGDDLII

SEQ ID NO: 1566 - protein, 9 aa, synthetic construct
GGQGADTLI

SEQ ID NO: 1567 - protein, 9 aa, synthetic construct
GGSGNDTLK

SEQ ID NO: 1568 - protein, 9 aa, synthetic construct
GGEGDDVLD

SEQ ID NO: 1569 - protein, 9 aa, synthetic construct
GGSGNDSLL

SEQ ID NO: 1570 - protein, 9 aa, synthetic construct
GGVGNDTLV

SEQ ID NO: 1571 - protein, 9 aa, synthetic construct
GGTGADSLT

SEQ ID NO: 1572 - protein, 9 aa, synthetic construct
GGAGSDVLD

SEQ ID NO: 1573 - protein, 9 aa, synthetic construct
GGAGDDLID

SEQ ID NO: 1574 - protein, 9 aa, synthetic construct
GGSGTDTAS

SEQ ID NO: 1575 - protein, 9 aa, synthetic construct
GGFGFDRLN

SEQ ID NO: 1576 - protein, 9 aa, synthetic construct
GGSGNDRLV

SEQ ID NO: 1577 - protein, 9 aa, synthetic construct
GGSGNDRLN

SEQ ID NO: 1578 - protein, 9 aa, synthetic construct
GGAGDDIFV

SEQ ID NO: 1579 - protein, 9 aa, synthetic construct
GGLGDDTLL

SEQ ID NO: 1580 - protein, 9 aa, synthetic construct
GGVGNDRLD

SEQ ID NO: 1581 - protein, 9 aa, synthetic construct
GGSGNDTII

SEQ ID NO: 1582 - protein, 9 aa, synthetic construct
GGAGNDHLY

SEQ ID NO: 1583 - protein, 9 aa, synthetic construct
GGQGDDTID

SEQ ID NO: 1584 - protein, 9 aa, synthetic construct
GGDGDDVLE

SEQ ID NO: 1585 - protein, 9 aa, synthetic construct
GGYGNDVYR

SEQ ID NO: 1586 - protein, 9 aa, synthetic construct
GGEGDDHLE

SEQ ID NO: 1587 - protein, 9 aa, synthetic construct
GGTGDDILD

SEQ ID NO: 1588 - protein, 9 aa, synthetic construct
GGAGSDTID

SEQ ID NO: 1589 - protein, 9 aa, synthetic construct
GGKGNDAYG

SEQ ID NO: 1590 - protein, 9 aa, synthetic construct
GGAGNDTVD

SEQ ID NO: 1591 - protein, 9 aa, synthetic construct
GGPGNDTLL

SEQ ID NO: 1592 - protein, 9 aa, synthetic construct
GGNGDDVLN

SEQ ID NO: 1593 - protein, 9 aa, synthetic construct
GGTGNDTYL

SEQ ID NO: 1594 - protein, 9 aa, synthetic construct
GGDGDDFLV

SEQ ID NO: 1595 - protein, 9 aa, synthetic construct
GGGGDDYLY

SEQ ID NO: 1596 - protein, 9 aa, synthetic construct
GGAGADSLN

SEQ ID NO: 1597 - protein, 9 aa, synthetic construct
GGFGNDILT

SEQ ID NO: 1598 - protein, 9 aa, synthetic construct
GGGGQDTLW

SEQ ID NO: 1599 - protein, 9 aa, synthetic construct
GGGGADLLI

SEQ ID NO: 1600 - protein, 9 aa, synthetic construct
GGSGNDWLD

SEQ ID NO: 1601 - protein, 9 aa, synthetic construct
GGSGNDYLY

SEQ ID NO: 1602 - protein, 9 aa, synthetic construct
GGAGGDVII

SEQ ID NO: 1603 - protein, 9 aa, synthetic construct
GGEGDDRLD

SEQ ID NO: 1604 - protein, 9 aa, synthetic construct
GGLGNDTLK

SEQ ID NO: 1605 - protein, 9 aa, synthetic construct
GGIGADTLT

SEQ ID NO: 1606 - protein, 9 aa, synthetic construct
GGTGSDTFV

SEQ ID NO: 1607 - protein, 9 aa, synthetic construct
GGGGGDILK

SEQ ID NO: 1608 - protein, 9 aa, synthetic construct
GGAGNDQLS

SEQ ID NO: 1609 - protein, 9 aa, synthetic construct
GGDGNDVLQ

SEQ ID NO: 1610 - protein, 9 aa, synthetic construct
GGEGEDLFK

SEQ ID NO: 1611 - protein, 9 aa, synthetic construct
GGKGDDILS

SEQ ID NO: 1612 - protein, 9 aa, synthetic construct
GGAGNDWLN

SEQ ID NO: 1613 - protein, 9 aa, synthetic construct
GGDGDDILE

SEQ ID NO: 1614 - protein, 9 aa, synthetic construct
GGGGDDVLV

SEQ ID NO: 1615 - protein, 9 aa, synthetic construct
GGEGYDRLS

SEQ ID NO: 1616 - protein, 9 aa, synthetic construct
GGAGNDVMT

SEQ ID NO: 1617 - protein, 9 aa, synthetic construct
GGDGDDSLF

SEQ ID NO: 1618 - protein, 9 aa, synthetic construct
GGTGNDELQ

SEQ ID NO: 1619 - protein, 9 aa, synthetic construct
GGAGADNLD

SEQ ID NO: 1620 - protein, 9 aa, synthetic construct
GGAGNDYLL

SEQ ID NO: 1621 - protein, 9 aa, synthetic construct
GGAGADRID

SEQ ID NO: 1622 - protein, 9 aa, synthetic construct
GGEGNDLLS

SEQ ID NO: 1623 - protein, 9 aa, synthetic construct
GGRGNDYLE

SEQ ID NO: 1624 - protein, 9 aa, synthetic construct
GGDGDDILT

SEQ ID NO: 1625 - protein, 9 aa, synthetic construct
GGTGNDSLL

SEQ ID NO: 1626 - protein, 9 aa, synthetic construct
GGTGNDSLV

SEQ ID NO: 1627 - protein, 9 aa, synthetic construct
GGAGEDVLI

SEQ ID NO: 1628 - protein, 9 aa, synthetic construct
GGTGNDTIS

SEQ ID NO: 1629 - protein, 9 aa, synthetic construct
GGDGDDYLY

SEQ ID NO: 1630 - protein, 9 aa, synthetic construct
GGAGRDSLT

SEQ ID NO: 1631 - protein, 9 aa, synthetic construct
GGAGDDSLA

SEQ ID NO: 1632 - protein, 9 aa, synthetic construct
GGGGADRLL

SEQ ID NO: 1633 - protein, 9 aa, synthetic construct
GGAGSDDLR

SEQ ID NO: 1634 - protein, 9 aa, synthetic construct
GGTGDDTIY

SEQ ID NO: 1635 - protein, 9 aa, synthetic construct
GGKGNDIIW

SEQ ID NO: 1636 - protein, 9 aa, synthetic construct
GGTGNDTFV

SEQ ID NO: 1637 - protein, 9 aa, synthetic construct
GGRGNDVLT

SEQ ID NO: 1638 - protein, 9 aa, synthetic construct
GGEGIDTAD

SEQ ID NO: 1639 - protein, 9 aa, synthetic construct
GGTGSDKFQ

SEQ ID NO: 1640 - protein, 9 aa, synthetic construct
GGAGNDKLF

SEQ ID NO: 1641 - protein, 9 aa, synthetic construct
GGTGNDRLT

SEQ ID NO: 1642 - protein, 9 aa, synthetic construct
GGVGNDTLL

SEQ ID NO: 1643 - protein, 9 aa, synthetic construct
GGAGRDRLE

SEQ ID NO: 1644 - protein, 9 aa, synthetic construct
GGLGNDIYY

SEQ ID NO: 1645 - protein, 9 aa, synthetic construct
GGAGDDDLR

SEQ ID NO: 1646 - protein, 9 aa, synthetic construct
GGSGDDRLS

SEQ ID NO: 1647 - protein, 9 aa, synthetic construct
GGNGNDSLL

SEQ ID NO: 1648 - protein, 9 aa, synthetic construct
GGDGNDVIN

SEQ ID NO: 1649 - protein, 9 aa, synthetic construct
GGDGDDSLY

SEQ ID NO: 1650 - protein, 9 aa, synthetic construct
GGNGTDTLI

SEQ ID NO: 1651 - protein, 9 aa, synthetic construct
GGDGTDTAV

SEQ ID NO: 1652 - protein, 9 aa, synthetic construct
GGKGSDTLT

SEQ ID NO: 1653 - protein, 9 aa, synthetic construct
GGSGSDVLD

SEQ ID NO: 1654 - protein, 9 aa, synthetic construct
GGSGNDQLF

SEQ ID NO: 1655 - protein, 9 aa, synthetic construct
GGPGNDTLE

SEQ ID NO: 1656 - protein, 9 aa, synthetic construct
GGAGDDRID

SEQ ID NO: 1657 - protein, 9 aa, synthetic construct
GGRGNDRLS

SEQ ID NO: 1658 - protein, 9 aa, synthetic construct
GGTGNDTIL

SEQ ID NO: 1659 - protein, 9 aa, synthetic construct
GGDGNDTYI

SEQ ID NO: 1660 - protein, 9 aa, synthetic construct
GGDGDDFVN

SEQ ID NO: 1661 - protein, 9 aa, synthetic construct
GGAGADRMT

SEQ ID NO: 1662 - protein, 9 aa, synthetic construct
GGKGDDILT

SEQ ID NO: 1663 - protein, 9 aa, synthetic construct
GGTGNDVLR

SEQ ID NO: 1664 - protein, 9 aa, synthetic construct
GGSGNDYLD

SEQ ID NO: 1665 - protein, 9 aa, synthetic construct
GGAGNDALT

SEQ ID NO: 1666 - protein, 9 aa, synthetic construct
GGAGADSMA

SEQ ID NO: 1667 - protein, 9 aa, synthetic construct
GGAGADRLA

SEQ ID NO: 1668 - protein, 9 aa, synthetic construct
GGAGRDYLD

SEQ ID NO: 1669 - protein, 9 aa, synthetic construct
GGAGSDSLS

SEQ ID NO: 1670 - protein, 9 aa, synthetic construct
GGLGNDVIY

SEQ ID NO: 1671 - protein, 9 aa, synthetic construct
GGQGTDYLV

SEQ ID NO: 1672 - protein, 9 aa, synthetic construct
GGGGRDLLQ

SEQ ID NO: 1673 - protein, 9 aa, synthetic construct
GGSGNDVLF

SEQ ID NO: 1674 - protein, 9 aa, synthetic construct
GGAGADILY

SEQ ID NO: 1675 - protein, 9 aa, synthetic construct
GGTGDDSLD

SEQ ID NO: 1676 - protein, 9 aa, synthetic construct
GGAGVDTLR

SEQ ID NO: 1677 - protein, 9 aa, synthetic construct
GGAGNDLFY

SEQ ID NO: 1678 - protein, 9 aa, synthetic construct
GGGGNDILT

SEQ ID NO: 1679 - protein, 9 aa, synthetic construct
GGEGDDGLA

SEQ ID NO: 1680 - protein, 9 aa, synthetic construct
GGSGDDVID

SEQ ID NO: 1681 - protein, 9 aa, synthetic construct
GGLGNDLLN

SEQ ID NO: 1682 - protein, 9 aa, synthetic construct
GGDGNDRIR

SEQ ID NO: 1683 - protein, 9 aa, synthetic construct
GGAGNDAIN

SEQ ID NO: 1684 - protein, 9 aa, synthetic construct
GGDGNDYLS

SEQ ID NO: 1685 - protein, 9 aa, synthetic construct
GGNGADSLS

SEQ ID NO: 1686 - protein, 9 aa, synthetic construct
GGGGNDYLA

SEQ ID NO: 1687 - protein, 9 aa, synthetic construct
GGTGDDVLN

SEQ ID NO: 1688 - protein, 9 aa, synthetic construct
GGGGNDRLI

SEQ ID NO: 1689 - protein, 9 aa, synthetic construct
GGTGLDKLY

SEQ ID NO: 1690 - protein, 9 aa, synthetic construct
GGGGNDRLL

SEQ ID NO: 1691 - protein, 9 aa, synthetic construct
GGAGNDTYR

SEQ ID NO: 1692 - protein, 9 aa, synthetic construct
GGDGIDQLF

SEQ ID NO: 1693 - protein, 9 aa, synthetic construct
GGLGDDRLD

SEQ ID NO: 1694 - protein, 9 aa, synthetic construct
GGAGKDTFV

SEQ ID NO: 1695 - protein, 9 aa, synthetic construct
GGNGHDTLR

SEQ ID NO: 1696 - protein, 9 aa, synthetic construct
GGLGDDTLV

SEQ ID NO: 1697 - protein, 9 aa, synthetic construct
GGTGADTLY

SEQ ID NO: 1698 - protein, 9 aa, synthetic construct
GGLGADTFK

SEQ ID NO: 1699 - protein, 9 aa, synthetic construct
GGAGGDRFE

SEQ ID NO: 1700 - protein, 9 aa, synthetic construct
GGRGDDTLI

SEQ ID NO: 1701 - protein, 9 aa, synthetic construct
GGTGNDVMA

SEQ ID NO: 1702 - protein, 9 aa, synthetic construct
GGTGADSMA

SEQ ID NO: 1703 - protein, 9 aa, synthetic construct
GGAGSDTLA

SEQ ID NO: 1704 - protein, 9 aa, synthetic construct
GGAGNDALH

SEQ ID NO: 1705 - protein, 9 aa, synthetic construct
GGAGGDVLN

SEQ ID NO: 1706 - protein, 9 aa, synthetic construct
GGKGNDYIY

SEQ ID NO: 1707 - protein, 9 aa, synthetic construct
GGGGSDLFI

SEQ ID NO: 1708 - protein, 9 aa, synthetic construct
GGNGADLLI

SEQ ID NO: 1709 - protein, 9 aa, synthetic construct
GGSGNDTIL

SEQ ID NO: 1710 - protein, 9 aa, synthetic construct
GGLGTDTLT

SEQ ID NO: 1711 - protein, 9 aa, synthetic construct
GGDGNDTLM

SEQ ID NO: 1712 - protein, 9 aa, synthetic construct
GGLGKDTFV

SEQ ID NO: 1713 - protein, 9 aa, synthetic construct
GGAGRDTLN

SEQ ID NO: 1714 - protein, 9 aa, synthetic construct
GGVGNDRLF

SEQ ID NO: 1715 - protein, 9 aa, synthetic construct
GGDGNDSLF

SEQ ID NO: 1716 - protein, 9 aa, synthetic construct
GGQGSDMLR

SEQ ID NO: 1717 - protein, 9 aa, synthetic construct
GGDGDDILA

SEQ ID NO: 1718 - protein, 9 aa, synthetic construct
GGGGGDTFV

SEQ ID NO: 1719 - protein, 9 aa, synthetic construct
GGEGNDSLL

SEQ ID NO: 1720 - protein, 9 aa, synthetic construct
GGTGADTMI

SEQ ID NO: 1721 - protein, 9 aa, synthetic construct
GGAGTDTLA

SEQ ID NO: 1722 - protein, 9 aa, synthetic construct
GGDGADSLS

SEQ ID NO: 1723 - protein, 9 aa, synthetic construct
GGDGDDTIE

SEQ ID NO: 1724 - protein, 9 aa, synthetic construct
GGYGKDTII

SEQ ID NO: 1725 - protein, 9 aa, synthetic construct
GGAGVDVLN

SEQ ID NO: 1726 - protein, 9 aa, synthetic construct
GGGGADRLI

SEQ ID NO: 1727 - protein, 9 aa, synthetic construct
GGAGDDLFL

SEQ ID NO: 1728 - protein, 9 aa, synthetic construct
GGLGADTLY

SEQ ID NO: 1729 - protein, 9 aa, synthetic construct
GGDGIDTVD

SEQ ID NO: 1730 - protein, 9 aa, synthetic construct
GGAGADVLV

SEQ ID NO: 1731 - protein, 9 aa, synthetic construct
GGFGQDTMT

SEQ ID NO: 1732 - protein, 9 aa, synthetic construct
GGEGNDVLT

SEQ ID NO: 1733 - protein, 9 aa, synthetic construct
GGNGADHLW

SEQ ID NO: 1734 - protein, 9 aa, synthetic construct
GGDGDDTII

SEQ ID NO: 1735 - protein, 9 aa, synthetic construct
GGAGADLLE

SEQ ID NO: 1736 - protein, 9 aa, synthetic construct
GGDGDDRLL

SEQ ID NO: 1737 - protein, 9 aa, synthetic construct
GGAGNDRIY

SEQ ID NO: 1738 - protein, 9 aa, synthetic construct
GGSGSDTLD

SEQ ID NO: 1739 - protein, 9 aa, synthetic construct
GGWGNDMLD

SEQ ID NO: 1740 - protein, 9 aa, synthetic construct
GGTGNDTMT

SEQ ID NO: 1741 - protein, 9 aa, synthetic construct
GGLGADIFI

SEQ ID NO: 1742 - protein, 9 aa, synthetic construct
GGEGIDGLR

SEQ ID NO: 1743 - protein, 9 aa, synthetic construct
GGRGDDRLL

SEQ ID NO: 1744 - protein, 9 aa, synthetic construct
GGSGRDTFV

SEQ ID NO: 1745 - protein, 9 aa, synthetic construct
GGSGNDTYY

SEQ ID NO: 1746 - protein, 9 aa, synthetic construct
GGRGSDLLD

SEQ ID NO: 1747 - protein, 9 aa, synthetic construct
GGTGNDLLN

SEQ ID NO: 1748 - protein, 9 aa, synthetic construct
GGAGDDRLV

SEQ ID NO: 1749 - protein, 9 aa, synthetic construct
GGDGNDRMA

SEQ ID NO: 1750 - protein, 9 aa, synthetic construct
GGIGNDTLL

SEQ ID NO: 1751 - protein, 9 aa, synthetic construct
GGEGDDTLN

SEQ ID NO: 1752 - protein, 9 aa, synthetic construct
GGAGNDTIG

SEQ ID NO: 1753 - protein, 9 aa, synthetic construct
GGAGADTMR

SEQ ID NO: 1754 - protein, 9 aa, synthetic construct
GGQGDDILH

SEQ ID NO: 1755 - protein, 9 aa, synthetic construct
GGAGADKLL

SEQ ID NO: 1756 - protein, 9 aa, synthetic construct
GGPGNDTLD

SEQ ID NO: 1757 - protein, 9 aa, synthetic construct
GGAGNDIIT

SEQ ID NO: 1758 - protein, 9 aa, synthetic construct
GGSGNDLLR

SEQ ID NO: 1759 - protein, 9 aa, synthetic construct
GGSGDDSLF

SEQ ID NO: 1760 - protein, 9 aa, synthetic construct
GGNGNDRLL

SEQ ID NO: 1761 - protein, 9 aa, synthetic construct
GGGGDDWII

SEQ ID NO: 1762 - protein, 9 aa, synthetic construct
GGAGDDVLH

SEQ ID NO: 1763 - protein, 9 aa, synthetic construct
GGEGDDILR

SEQ ID NO: 1764 - protein, 9 aa, synthetic construct
GGDGNDALD

SEQ ID NO: 1765 - protein, 9 aa, synthetic construct
GGDGADRLD

SEQ ID NO: 1766 - protein, 9 aa, synthetic construct
GGSGNDKLF

SEQ ID NO: 1767 - protein, 9 aa, synthetic construct
GGSGIDQLS

SEQ ID NO: 1768 - protein, 9 aa, synthetic construct
GGAGADLFI

SEQ ID NO: 1769 - protein, 9 aa, synthetic construct
GGAGADLFR

SEQ ID NO: 1770 - protein, 9 aa, synthetic construct
GGEGFDYIE

SEQ ID NO: 1771 - protein, 9 aa, synthetic construct
GGAGNDMLL

SEQ ID NO: 1772 - protein, 9 aa, synthetic construct
GGDGNDHLV

SEQ ID NO: 1773 - protein, 9 aa, synthetic construct
GGAGRDTAS

SEQ ID NO: 1774 - protein, 9 aa, synthetic construct
GGAGADTLH

SEQ ID NO: 1775 - protein, 9 aa, synthetic construct
GGVGADTMI

SEQ ID NO: 1776 - protein, 9 aa, synthetic construct
GGTGADGLI

SEQ ID NO: 1777 - protein, 9 aa, synthetic construct
GGGGNDVLS

SEQ ID NO: 1778 - protein, 9 aa, synthetic construct
GGDGNDSLT

SEQ ID NO: 1779 - protein, 9 aa, synthetic construct
GGAGHDTLI

SEQ ID NO: 1780 - protein, 9 aa, synthetic construct
GGIGHDTME

SEQ ID NO: 1781 - protein, 9 aa, synthetic construct
GGAGSDKLT

SEQ ID NO: 1782 - protein, 9 aa, synthetic construct
GGEGDDILL

SEQ ID NO: 1783 - protein, 9 aa, synthetic construct
GGAGNDSIL

SEQ ID NO: 1784 - protein, 9 aa, synthetic construct
GGLGNDSYI

SEQ ID NO: 1785 - protein, 9 aa, synthetic construct
GGLGDDVLN

SEQ ID NO: 1786 - protein, 9 aa, synthetic construct
GGTGNDFLD

SEQ ID NO: 1787 - protein, 9 aa, synthetic construct
GGSGADRLI

SEQ ID NO: 1788 - protein, 9 aa, synthetic construct
GGAGKDTLI

SEQ ID NO: 1789 - protein, 9 aa, synthetic construct
GGAGNDTVL

SEQ ID NO: 1790 - protein, 9 aa, synthetic construct
GGLGEDTMI

SEQ ID NO: 1791 - protein, 9 aa, synthetic construct
GGPGADTLL

SEQ ID NO: 1792 - protein, 9 aa, synthetic construct
GGAGNDLIS

SEQ ID NO: 1793 - protein, 9 aa, synthetic construct
GGSGDDFLI

SEQ ID NO: 1794 - protein, 9 aa, synthetic construct
GGTGNDVLI

SEQ ID NO: 1795 - protein, 9 aa, synthetic construct
GGAGIDKMS

SEQ ID NO: 1796 - protein, 9 aa, synthetic construct
GGRGQDALF

SEQ ID NO: 1797 - protein, 9 aa, synthetic construct
GGAGNDSLH

SEQ ID NO: 1798 - protein, 9 aa, synthetic construct
GGEGADILV

SEQ ID NO: 1799 - protein, 9 aa, synthetic construct
GGQGFDILT

SEQ ID NO: 1800 - protein, 9 aa, synthetic construct
GGSGNDTMR

SEQ ID NO: 1801 - protein, 9 aa, synthetic construct
GGTGNDRLI

SEQ ID NO: 1802 - protein, 9 aa, synthetic construct
GGAGADLID

SEQ ID NO: 1803 - protein, 9 aa, synthetic construct
GGLGADALD

SEQ ID NO: 1804 - protein, 9 aa, synthetic construct
GGAGADAFV

SEQ ID NO: 1805 - protein, 9 aa, synthetic construct
GGRGNDTLT

SEQ ID NO: 1806 - protein, 9 aa, synthetic construct
GGEGNDRLE

SEQ ID NO: 1807 - protein, 9 aa, synthetic construct
GGDGNDLLN

SEQ ID NO: 1808 - protein, 9 aa, synthetic construct
GGAGDDRLR

SEQ ID NO: 1809 - protein, 9 aa, synthetic construct
GGVGNDTLM

SEQ ID NO: 1810 - protein, 9 aa, synthetic construct
GGFGHDRIN

SEQ ID NO: 1811 - protein, 9 aa, synthetic construct
GGVGDDTLT

SEQ ID NO: 1812 - protein, 9 aa, synthetic construct
GGAGNDTMA

SEQ ID NO: 1813 - protein, 9 aa, synthetic construct
GGAGDDELI

SEQ ID NO: 1814 - protein, 9 aa, synthetic construct
GGGGNDMLD

SEQ ID NO: 1815 - protein, 9 aa, synthetic construct
GGGGDDTID

SEQ ID NO: 1816 - protein, 9 aa, synthetic construct
GGDGDDLLV

SEQ ID NO: 1817 - protein, 9 aa, synthetic construct
GGNGADTFV

SEQ ID NO: 1818 - protein, 9 aa, synthetic construct
GGAGNDSLR

SEQ ID NO: 1819 - protein, 9 aa, synthetic construct
GGAGNDVIT

SEQ ID NO: 1820 - protein, 9 aa, synthetic construct
GGSGADTFR

SEQ ID NO: 1821 - protein, 9 aa, synthetic construct
GGKGDDRMS

SEQ ID NO: 1822 - protein, 9 aa, synthetic construct
GGNGNDRLF

SEQ ID NO: 1823 - protein, 9 aa, synthetic construct
GGAGNDSLQ

SEQ ID NO: 1824 - protein, 9 aa, synthetic construct
GGSGNDSLT

SEQ ID NO: 1825 - protein, 9 aa, synthetic construct
GGTGDDILI

SEQ ID NO: 1826 - protein, 9 aa, synthetic construct
GGTGDDTLF

SEQ ID NO: 1827 - protein, 9 aa, synthetic construct
GGAGIDTMI

SEQ ID NO: 1828 - protein, 9 aa, synthetic construct
GGNGNDKLY

SEQ ID NO: 1829 - protein, 9 aa, synthetic construct
GGGGNDSLS

SEQ ID NO: 1830 - protein, 9 aa, synthetic construct
GGGGADTLF

SEQ ID NO: 1831 - protein, 9 aa, synthetic construct
GGYGNDYLD

SEQ ID NO: 1832 - protein, 9 aa, synthetic construct
GGGGNDVIY

SEQ ID NO: 1833 - protein, 9 aa, synthetic construct
GGAGNDQMQ

SEQ ID NO: 1834 - protein, 9 aa, synthetic construct
GGLGNDTLA

SEQ ID NO: 1835 - protein, 9 aa, synthetic construct
GGAGVDTAS

SEQ ID NO: 1836 - protein, 9 aa, synthetic construct
GGEGRDILD

SEQ ID NO: 1837 - protein, 9 aa, synthetic construct
GGLGNDTLF

SEQ ID NO: 1838 - protein, 9 aa, synthetic construct
GGKGADTLT

SEQ ID NO: 1839 - protein, 9 aa, synthetic construct
GGAGDDWLD

SEQ ID NO: 1840 - protein, 9 aa, synthetic construct
GGDGDDTIL

SEQ ID NO: 1841 - protein, 9 aa, synthetic construct
GGDGDDLIS

SEQ ID NO: 1842 - protein, 9 aa, synthetic construct
GGTGSDIFV

SEQ ID NO: 1843 - protein, 9 aa, synthetic construct
GGDGDDFID

SEQ ID NO: 1844 - protein, 9 aa, synthetic construct
GGSGNDQLI

SEQ ID NO: 1845 - protein, 9 aa, synthetic construct
GGSGNDILF

SEQ ID NO: 1846 - protein, 9 aa, synthetic construct
GGRGDDILT

SEQ ID NO: 1847 - protein, 9 aa, synthetic construct
GGLGIDTLI

SEQ ID NO: 1848 - protein, 9 aa, synthetic construct
GGAGDDNLR

SEQ ID NO: 1849 - protein, 9 aa, synthetic construct
GGEGNDILF

SEQ ID NO: 1850 - protein, 9 aa, synthetic construct
GGQGNDMMT

SEQ ID NO: 1851 - protein, 9 aa, synthetic construct
GGAGDDMLI

SEQ ID NO: 1852 - protein, 9 aa, synthetic construct
GGAGADVFI

SEQ ID NO: 1853 - protein, 9 aa, synthetic construct
GGEGDDSLD

SEQ ID NO: 1854 - protein, 9 aa, synthetic construct
GGGGSDTLL

SEQ ID NO: 1855 - protein, 9 aa, synthetic construct
GGGGADVFR

SEQ ID NO: 1856 - protein, 9 aa, synthetic construct
GGSGDDILF

SEQ ID NO: 1857 - protein, 9 aa, synthetic construct
GGDGYDVMI

SEQ ID NO: 1858 - protein, 9 aa, synthetic construct
GGAGNDQLQ

SEQ ID NO: 1859 - protein, 9 aa, synthetic construct
GGLGADTIA

SEQ ID NO: 1860 - protein, 9 aa, synthetic construct
GGNGNDVLN

SEQ ID NO: 1861 - protein, 9 aa, synthetic construct
GGLGADTIY

SEQ ID NO: 1862 - protein, 9 aa, synthetic construct
GGKGDDTYV

SEQ ID NO: 1863 - protein, 9 aa, synthetic construct
GGPGNDTLI

SEQ ID NO: 1864 - protein, 9 aa, synthetic construct
GGQGDDTLR

SEQ ID NO: 1865 - protein, 9 aa, synthetic construct
GGFGADTLD

SEQ ID NO: 1866 - protein, 9 aa, synthetic construct
GGLGNDLLI

SEQ ID NO: 1867 - protein, 9 aa, synthetic construct
GGAGSDVLI

SEQ ID NO: 1868 - protein, 9 aa, synthetic construct
GGSGADTLV

SEQ ID NO: 1869 - protein, 9 aa, synthetic construct
GGDGVDTAV

SEQ ID NO: 1870 - protein, 9 aa, synthetic construct
GGDGDDVIL

SEQ ID NO: 1871 - protein, 9 aa, synthetic construct
GGQGNDTLA

SEQ ID NO: 1872 - protein, 9 aa, synthetic construct
GGAGNDQLV

SEQ ID NO: 1873 - protein, 9 aa, synthetic construct
GGTGADTMR

SEQ ID NO: 1874 - protein, 9 aa, synthetic construct
GGDGDDSLV

SEQ ID NO: 1875 - protein, 9 aa, synthetic construct
GGGGNDLLY

SEQ ID NO: 1876 - protein, 9 aa, synthetic construct
GGAGNDWLE

SEQ ID NO: 1877 - protein, 9 aa, synthetic construct
GGSGADTMA

SEQ ID NO: 1878 - protein, 9 aa, synthetic construct
GGAGDDVLK

SEQ ID NO: 1879 - protein, 9 aa, synthetic construct
GGSGDDSLD

SEQ ID NO: 1880 - protein, 9 aa, synthetic construct
GGAGNDTIM

SEQ ID NO: 1881 - protein, 9 aa, synthetic construct
GGSGDDTYL

SEQ ID NO: 1882 - protein, 9 aa, synthetic construct
GGSGADVFR

SEQ ID NO: 1883 - protein, 9 aa, synthetic construct
GGAGDDVLQ

SEQ ID NO: 1884 - protein, 9 aa, synthetic construct
GGQGADTLS

SEQ ID NO: 1885 - protein, 9 aa, synthetic construct
GGGGNDLLN

SEQ ID NO: 1886 - protein, 9 aa, synthetic construct
GGDGNDIIY

SEQ ID NO: 1887 - protein, 9 aa, synthetic construct
GGAGKDTLV

SEQ ID NO: 1888 - protein, 9 aa, synthetic construct
GGAGADLLL

SEQ ID NO: 1889 - protein, 9 aa, synthetic construct
GGNGADTFK

SEQ ID NO: 1890 - protein, 9 aa, synthetic construct
GGSGDDTFI

SEQ ID NO: 1891 - protein, 9 aa, synthetic construct
GGGGKDSLM

SEQ ID NO: 1892 - protein, 9 aa, synthetic construct
GGFGNDTYR

SEQ ID NO: 1893 - protein, 9 aa, synthetic construct
GGAGADVFL

SEQ ID NO: 1894 - protein, 9 aa, synthetic construct
GGDGDDSIL

SEQ ID NO: 1895 - protein, 9 aa, synthetic construct
GGSGADLLD

SEQ ID NO: 1896 - protein, 9 aa, synthetic construct
GGEGFDTVS

SEQ ID NO: 1897 - protein, 9 aa, synthetic construct
GGAGNDELH

SEQ ID NO: 1898 - protein, 9 aa, synthetic construct
GGNGADTLN

SEQ ID NO: 1899 - protein, 9 aa, synthetic construct
GGDGNDTIR

SEQ ID NO: 1900 - protein, 9 aa, synthetic construct
GGSGDDTLA

SEQ ID NO: 1901 - protein, 9 aa, synthetic construct
GGDGNDYLF

SEQ ID NO: 1902 - protein, 9 aa, synthetic construct
GGKGDDFLS

SEQ ID NO: 1903 - protein, 9 aa, synthetic construct
GGLGNDRLF

SEQ ID NO: 1904 - protein, 9 aa, synthetic construct
GGDGNDLIN

SEQ ID NO: 1905 - protein, 9 aa, synthetic construct
GGGGADTIY

SEQ ID NO: 1906 - protein, 9 aa, synthetic construct
GGSGADIFR

SEQ ID NO: 1907 - protein, 9 aa, synthetic construct
GGAGNDIIV

SEQ ID NO: 1908 - protein, 9 aa, synthetic construct
GGDGNDTII

SEQ ID NO: 1909 - protein, 9 aa, synthetic construct
GGEGADRLI

SEQ ID NO: 1910 - protein, 9 aa, synthetic construct
GGVGNDSLD

SEQ ID NO: 1911 - protein, 9 aa, synthetic construct
GGDGFDTFV

SEQ ID NO: 1912 - protein, 9 aa, synthetic construct
GGTGADKLT

SEQ ID NO: 1913 - protein, 9 aa, synthetic construct
GGQGNDTLL

SEQ ID NO: 1914 - protein, 9 aa, synthetic construct
GGAGNDVYY

SEQ ID NO: 1915 - protein, 9 aa, synthetic construct
GGDGADVFV

SEQ ID NO: 1916 - protein, 9 aa, synthetic construct
GGSGSDTLI

SEQ ID NO: 1917 - protein, 9 aa, synthetic construct
GGSGSDVFV

SEQ ID NO: 1918 - protein, 9 aa, synthetic construct
GGSGNDMLY

SEQ ID NO: 1919 - protein, 9 aa, synthetic construct
GGAGIDTLV

SEQ ID NO: 1920 - protein, 9 aa, synthetic construct
GGDGNDSLI

SEQ ID NO: 1921 - protein, 9 aa, synthetic construct
GGAGNDYLY

SEQ ID NO: 1922 - protein, 9 aa, synthetic construct
GGGGADTFD

SEQ ID NO: 1923 - protein, 9 aa, synthetic construct
GGSGIDTAV

SEQ ID NO: 1924 - protein, 9 aa, synthetic construct
GGEGDDLLS

SEQ ID NO: 1925 - protein, 9 aa, synthetic construct
GGTGSDKLY

SEQ ID NO: 1926 - protein, 9 aa, synthetic construct
GGSGDDVLA

SEQ ID NO: 1927 - protein, 9 aa, synthetic construct
GGAGGDSLD

SEQ ID NO: 1928 - protein, 9 aa, synthetic construct
GGGGNDWLY

SEQ ID NO: 1929 - protein, 9 aa, synthetic construct
GGEGIDTVV

SEQ ID NO: 1930 - protein, 9 aa, synthetic construct
GGDGDDMLF

SEQ ID NO: 1931 - protein, 9 aa, synthetic construct
GGAGDDIYI

SEQ ID NO: 1932 - protein, 9 aa, synthetic construct
GGGGEDVLD

SEQ ID NO: 1933 - protein, 9 aa, synthetic construct
GGTGHDTIA

SEQ ID NO: 1934 - protein, 9 aa, synthetic construct
GGTGDDIYV

SEQ ID NO: 1935 - protein, 9 aa, synthetic construct
GGAGNDRLR

SEQ ID NO: 1936 - protein, 9 aa, synthetic construct
GGFGSDTMT

SEQ ID NO: 1937 - protein, 9 aa, synthetic construct
GGTGNDTII

SEQ ID NO: 1938 - protein, 9 aa, synthetic construct
GGAGHDRLL

SEQ ID NO: 1939 - protein, 9 aa, synthetic construct
GGAGKDFLL

SEQ ID NO: 1940 - protein, 9 aa, synthetic construct
GGAGVDTLK

SEQ ID NO: 1941 - protein, 9 aa, synthetic construct
GGTGADTFA

SEQ ID NO: 1942 - protein, 9 aa, synthetic construct
GGSGDDVLS

SEQ ID NO: 1943 - protein, 9 aa, synthetic construct
GGAGDDKVE

SEQ ID NO: 1944 - protein, 9 aa, synthetic construct
GGAGDDALT

SEQ ID NO: 1945 - protein, 9 aa, synthetic construct
GGSGNDILL

SEQ ID NO: 1946 - protein, 9 aa, synthetic construct
GGAGNDSLE

SEQ ID NO: 1947 - protein, 9 aa, synthetic construct
GGAGADSID

SEQ ID NO: 1948 - protein, 9 aa, synthetic construct
GGRGKDRLA

SEQ ID NO: 1949 - protein, 9 aa, synthetic construct
GGTGNDMYR

SEQ ID NO: 1950 - protein, 9 aa, synthetic construct
GGEGNDFLA

SEQ ID NO: 1951 - protein, 9 aa, synthetic construct
GGAGSDTYV

SEQ ID NO: 1952 - protein, 9 aa, synthetic construct
GGGGSDVFV

SEQ ID NO: 1953 - protein, 9 aa, synthetic construct
GGGGNDTYI

SEQ ID NO: 1954 - protein, 9 aa, synthetic construct
GGAGSDTYL

SEQ ID NO: 1955 - protein, 9 aa, synthetic construct
GGLGADRLR

SEQ ID NO: 1956 - protein, 9 aa, synthetic construct
GGGGSDILT

SEQ ID NO: 1957 - protein, 9 aa, synthetic construct
GGAGNDALI

SEQ ID NO: 1958 - protein, 9 aa, synthetic construct
GGLGADSLT

SEQ ID NO: 1959 - protein, 9 aa, synthetic construct
GGAGHDYLN

SEQ ID NO: 1960 - protein, 9 aa, synthetic construct
GGIGDDIFK

SEQ ID NO: 1961 - protein, 9 aa, synthetic construct
GGAGSDILT

SEQ ID NO: 1962 - protein, 9 aa, synthetic construct
GGAGSDHLY

SEQ ID NO: 1963 - protein, 9 aa, synthetic construct
GGDGSDTYV

SEQ ID NO: 1964 - protein, 9 aa, synthetic construct
GGAGHDLLD

SEQ ID NO: 1965 - protein, 9 aa, synthetic construct
GGSGSDTLT

SEQ ID NO: 1966 - protein, 9 aa, synthetic construct
GGKGADQLT

SEQ ID NO: 1967 - protein, 9 aa, synthetic construct
GGSGNDSID

SEQ ID NO: 1968 - protein, 9 aa, synthetic construct
GGSGNDLLN

SEQ ID NO: 1969 - protein, 9 aa, synthetic construct
GGEGSDVYR

SEQ ID NO: 1970 - protein, 9 aa, synthetic construct
GGTGDDLLA

SEQ ID NO: 1971 - protein, 9 aa, synthetic construct
GGEGNDILS

SEQ ID NO: 1972 - protein, 9 aa, synthetic construct
GGAGNDAID

SEQ ID NO: 1973 - protein, 9 aa, synthetic construct
GGTGDDLLD

SEQ ID NO: 1974 - protein, 9 aa, synthetic construct
GGSGDDTID

SEQ ID NO: 1975 - protein, 9 aa, synthetic construct
GGTGNDVMS

SEQ ID NO: 1976 - protein, 9 aa, synthetic construct
GGAGDDFIN

SEQ ID NO: 1977 - protein, 9 aa, synthetic construct
GGGGNDSLN

SEQ ID NO: 1978 - protein, 9 aa, synthetic construct
GGSGDDTLF

SEQ ID NO: 1979 - protein, 9 aa, synthetic construct
GGAGNDQLT

SEQ ID NO: 1980 - protein, 9 aa, synthetic construct
GGTGADTMT

SEQ ID NO: 1981 - protein, 9 aa, synthetic construct
GGEGADTLL

SEQ ID NO: 1982 - protein, 9 aa, synthetic construct
GGAGDDTII

SEQ ID NO: 1983 - protein, 9 aa, synthetic construct
GGTGTDTAS

SEQ ID NO: 1984 - protein, 9 aa, synthetic construct
GGEGDDTII

SEQ ID NO: 1985 - protein, 9 aa, synthetic construct
GGGGNDVIN

SEQ ID NO: 1986 - protein, 9 aa, synthetic construct
GGEGKDTLK

SEQ ID NO: 1987 - protein, 9 aa, synthetic construct
GGRGNDRLI

SEQ ID NO: 1988 - protein, 9 aa, synthetic construct
GGSGKDTLI

SEQ ID NO: 1989 - protein, 9 aa, synthetic construct
GGNGKDVFI

SEQ ID NO: 1990 - protein, 9 aa, synthetic construct
GGAGQDTLD

SEQ ID NO: 1991 - protein, 9 aa, synthetic construct
GGAGRDVLR

SEQ ID NO: 1992 - protein, 9 aa, synthetic construct
GGEGNDTIN

SEQ ID NO: 1993 - protein, 9 aa, synthetic construct
GGAGRDRLI

SEQ ID NO: 1994 - protein, 9 aa, synthetic construct
GGSGNDHLL

SEQ ID NO: 1995 - protein, 9 aa, synthetic construct
GGLGEDRLF

SEQ ID NO: 1996 - protein, 9 aa, synthetic construct
GGDGQDTLQ

SEQ ID NO: 1997 - protein, 9 aa, synthetic construct
GGAGNDTFK

SEQ ID NO: 1998 - protein, 9 aa, synthetic construct
GGTGSDTAS

SEQ ID NO: 1999 - protein, 9 aa, synthetic construct
GGTGNDRLS

SEQ ID NO: 2000 - protein, 9 aa, synthetic construct
GGAGNDTFL

SEQ ID NO: 2001 - protein, 9 aa, synthetic construct
GGLGADAMA

SEQ ID NO: 2002 - protein, 9 aa, synthetic construct
GGAGNDRFV

SEQ ID NO: 2003 - protein, 9 aa, synthetic construct
GGEGNDILD

SEQ ID NO: 2004 - protein, 9 aa, synthetic construct
GGDGDDILL

SEQ ID NO: 2005 - protein, 9 aa, synthetic construct
GGAGSDLLD

SEQ ID NO: 2006 - protein, 9 aa, synthetic construct
GGAGDDIIF

SEQ ID NO: 2007 - protein, 9 aa, synthetic construct
GGEGDDLLQ

SEQ ID NO: 2008 - protein, 9 aa, synthetic construct
GGTGNDQLF

SEQ ID NO: 2009 - protein, 9 aa, synthetic construct
GGDGSDTLI

SEQ ID NO: 2010 - protein, 9 aa, synthetic construct
GGFGSDRVN

SEQ ID NO: 2011 - protein, 9 aa, synthetic construct
GGAGQDTLS

SEQ ID NO: 2012 - protein, 9 aa, synthetic construct
GGDGNDLLY

SEQ ID NO: 2013 - protein, 9 aa, synthetic construct
GGAGDDVLM

SEQ ID NO: 2014 - protein, 9 aa, synthetic construct
GGEGNDLLY

SEQ ID NO: 2015 - protein, 9 aa, synthetic construct
GGIGNDTFV

SEQ ID NO: 2016 - protein, 9 aa, synthetic construct
GGTGNDLLT

SEQ ID NO: 2017 - protein, 9 aa, synthetic construct
GGDGNDIID

SEQ ID NO: 2018 - protein, 9 aa, synthetic construct
GGAGIDTLS

SEQ ID NO: 2019 - protein, 9 aa, synthetic construct
GGIGNDSLD

SEQ ID NO: 2020 - protein, 9 aa, synthetic construct
GGFGQDTLT

SEQ ID NO: 2021 - protein, 9 aa, synthetic construct
GGQGNDTIR

SEQ ID NO: 2022 - protein, 9 aa, synthetic construct
GGTGHDILS

SEQ ID NO: 2023 - protein, 9 aa, synthetic construct
GGRGADTLT

SEQ ID NO: 2024 - protein, 9 aa, synthetic construct
GGAGNDEIS

SEQ ID NO: 2025 - protein, 9 aa, synthetic construct
GGEGNDILN

SEQ ID NO: 2026 - protein, 9 aa, synthetic construct
GGIGNDVLI

SEQ ID NO: 2027 - protein, 9 aa, synthetic construct
GGAGNDLFV

SEQ ID NO: 2028 - protein, 9 aa, synthetic construct
GGKGNDKLY

SEQ ID NO: 2029 - protein, 9 aa, synthetic construct
GGGGQDQLF

SEQ ID NO: 2030 - protein, 9 aa, synthetic construct
GGQGNDTLM

SEQ ID NO: 2031 - protein, 9 aa, synthetic construct
GGAGNDVVA

SEQ ID NO: 2032 - protein, 9 aa, synthetic construct
GGVGADTLD

SEQ ID NO: 2033 - protein, 9 aa, synthetic construct
GGDGDDTYL

SEQ ID NO: 2034 - protein, 9 aa, synthetic construct
GGAGNDLYR

SEQ ID NO: 2035 - protein, 9 aa, synthetic construct
GGRGADVFV

SEQ ID NO: 2036 - protein, 9 aa, synthetic construct
GGSGNDRLL

SEQ ID NO: 2037 - protein, 9 aa, synthetic construct
GGAGDDVIH

SEQ ID NO: 2038 - protein, 9 aa, synthetic construct
GGSGNDLLQ

SEQ ID NO: 2039 - protein, 9 aa, synthetic construct
GGAGNDILH

SEQ ID NO: 2040 - protein, 9 aa, synthetic construct
GGIGRDQLR

SEQ ID NO: 2041 - protein, 9 aa, synthetic construct
GGQGDDTIL

SEQ ID NO: 2042 - protein, 9 aa, synthetic construct
GGLGSDTLD

SEQ ID NO: 2043 - protein, 9 aa, synthetic construct
GGEGADTLN

SEQ ID NO: 2044 - protein, 9 aa, synthetic construct
GGAGDDTIV

SEQ ID NO: 2045 - protein, 9 aa, synthetic construct
GGEGNDVLS

SEQ ID NO: 2046 - protein, 9 aa, synthetic construct
GGEGDDILY

SEQ ID NO: 2047 - protein, 9 aa, synthetic construct
GGDGADLIH

SEQ ID NO: 2048 - protein, 9 aa, synthetic construct
GGYGNDTLN

SEQ ID NO: 2049 - protein, 9 aa, synthetic construct
GGGGSDLIS

SEQ ID NO: 2050 - protein, 9 aa, synthetic construct
GGAGADILQ

SEQ ID NO: 2051 - protein, 9 aa, synthetic construct
GGEGEDALQ

SEQ ID NO: 2052 - protein, 9 aa, synthetic construct
GGLGNDTIT

SEQ ID NO: 2053 - protein, 9 aa, synthetic construct
GGNGNDTLV

SEQ ID NO: 2054 - protein, 9 aa, synthetic construct
GGDGADTIT

SEQ ID NO: 2055 - protein, 9 aa, synthetic construct
GGLGNDIYL

SEQ ID NO: 2056 - protein, 9 aa, synthetic construct
GGEGDDLID

SEQ ID NO: 2057 - protein, 9 aa, synthetic construct
GGDGEDMLA

SEQ ID NO: 2058 - protein, 9 aa, synthetic construct
GGAGADQLT

SEQ ID NO: 2059 - protein, 9 aa, synthetic construct
GGYGADTYI

SEQ ID NO: 2060 - protein, 9 aa, synthetic construct
GGAGADQFF

SEQ ID NO: 2061 - protein, 9 aa, synthetic construct
GGYGNDTYV

SEQ ID NO: 2062 - protein, 9 aa, synthetic construct
GGAGADTYV

SEQ ID NO: 2063 - protein, 9 aa, synthetic construct
GGYGNDYID

SEQ ID NO: 2064 - protein, 9 aa, synthetic construct
GGAGADRMV

SEQ ID NO: 2065 - protein, 9 aa, synthetic construct
GGDGADTIY

SEQ ID NO: 2066 - protein, 9 aa, synthetic construct
GGLGNDTMT

SEQ ID NO: 2067 - protein, 9 aa, synthetic construct
GGAGADLLN

SEQ ID NO: 2068 - protein, 9 aa, synthetic construct
GGAGKDTLA

SEQ ID NO: 2069 - protein, 9 aa, synthetic construct
GGKGDDVLI

SEQ ID NO: 2070 - protein, 9 aa, synthetic construct
GGLGNDVLS

SEQ ID NO: 2071 - protein, 9 aa, synthetic construct
GGDGYDALG

SEQ ID NO: 2072 - protein, 9 aa, synthetic construct
GGLGNDILM

SEQ ID NO: 2073 - protein, 9 aa, synthetic construct
GGAGADNLT

SEQ ID NO: 2074 - protein, 9 aa, synthetic construct
GGWGNDTLT

SEQ ID NO: 2075 - protein, 9 aa, synthetic construct
GGQGNDTLS

SEQ ID NO: 2076 - protein, 9 aa, synthetic construct
GGRGNDRLD

SEQ ID NO: 2077 - protein, 9 aa, synthetic construct
GGSGDDVLT

SEQ ID NO: 2078 - protein, 9 aa, synthetic construct
GGRGADRMK

SEQ ID NO: 2079 - protein, 9 aa, synthetic construct
GGKGHDALE

SEQ ID NO: 2080 - protein, 9 aa, synthetic construct
GGGGDDMLI

SEQ ID NO: 2081 - protein, 9 aa, synthetic construct
GGAGHDTFV

SEQ ID NO: 2082 - protein, 9 aa, synthetic construct
GGAGNDMLI

SEQ ID NO: 2083 - protein, 9 aa, synthetic construct
GGTGEDAIF

SEQ ID NO: 2084 - protein, 9 aa, synthetic construct
GGRGRDTLK

SEQ ID NO: 2085 - protein, 9 aa, synthetic construct
GGSGNDLIY

SEQ ID NO: 2086 - protein, 9 aa, synthetic construct
GGAGNDNLD

SEQ ID NO: 2087 - protein, 9 aa, synthetic construct
GGTGNDALY

SEQ ID NO: 2088 - protein, 9 aa, synthetic construct
GGSGADNMR

SEQ ID NO: 2089 - protein, 9 aa, synthetic construct
GGRGHDFLD

SEQ ID NO: 2090 - protein, 9 aa, synthetic construct
GGLGRDTLD

SEQ ID NO: 2091 - protein, 9 aa, synthetic construct
GGDGIDTAS

SEQ ID NO: 2092 - protein, 9 aa, synthetic construct
GGSGTDTLI

SEQ ID NO: 2093 - protein, 9 aa, synthetic construct
GGPGNDYLD

SEQ ID NO: 2094 - protein, 9 aa, synthetic construct
GGAGNDVIE

SEQ ID NO: 2095 - protein, 9 aa, synthetic construct
GGGGHDTLI

SEQ ID NO: 2096 - protein, 9 aa, synthetic construct
GGDGDDFIN

SEQ ID NO: 2097 - protein, 9 aa, synthetic construct
GGAGNDELD

SEQ ID NO: 2098 - protein, 9 aa, synthetic construct
GGLGADTMS

SEQ ID NO: 2099 - protein, 9 aa, synthetic construct
GGLGADTLL

SEQ ID NO: 2100 - protein, 9 aa, synthetic construct
GGVGNDSLN

SEQ ID NO: 2101 - protein, 9 aa, synthetic construct
GGAGNDKLL

SEQ ID NO: 2102 - protein, 9 aa, synthetic construct
GGAGADSLY

SEQ ID NO: 2103 - protein, 9 aa, synthetic construct
GGGGSDVLD

SEQ ID NO: 2104 - protein, 9 aa, synthetic construct
GGEGADTLY

SEQ ID NO: 2105 - protein, 9 aa, synthetic construct
GGLGNDVLK

SEQ ID NO: 2106 - protein, 9 aa, synthetic construct
GGAGNDMLN

SEQ ID NO: 2107 - protein, 9 aa, synthetic construct
GGYGNDTAS

SEQ ID NO: 2108 - protein, 9 aa, synthetic construct
GGDGFDVLS

SEQ ID NO: 2109 - protein, 9 aa, synthetic construct
GGAGADQLS

SEQ ID NO: 2110 - protein, 9 aa, synthetic construct
GGAGADQLF

SEQ ID NO: 2111 - protein, 9 aa, synthetic construct
GGAGLDKLT

SEQ ID NO: 2112 - protein, 9 aa, synthetic construct
GGAGVDTLS

SEQ ID NO: 2113 - protein, 9 aa, synthetic construct
GGAGNDTVN

SEQ ID NO: 2114 - protein, 9 aa, synthetic construct
GGEGNDTVD

SEQ ID NO: 2115 - protein, 9 aa, synthetic construct
GGDGNDTIH

SEQ ID NO: 2116 - protein, 9 aa, synthetic construct
GGDGNDNLD

SEQ ID NO: 2117 - protein, 9 aa, synthetic construct
GGLGDDFIE

SEQ ID NO: 2118 - protein, 9 aa, synthetic construct
GGAGTDSLT

SEQ ID NO: 2119 - protein, 9 aa, synthetic construct
GGAGRDSFV

SEQ ID NO: 2120 - protein, 9 aa, synthetic construct
GGDGNDALF

SEQ ID NO: 2121 - protein, 9 aa, synthetic construct
GGTGADTIY

SEQ ID NO: 2122 - protein, 9 aa, synthetic construct
GGSGADTMT

SEQ ID NO: 2123 - protein, 9 aa, synthetic construct
GGFGSDTVI

SEQ ID NO: 2124 - protein, 9 aa, synthetic construct
GGTGADRLD

SEQ ID NO: 2125 - protein, 9 aa, synthetic construct
GGGGDDSLD

SEQ ID NO: 2126 - protein, 9 aa, synthetic construct
GGAGDDLFF

SEQ ID NO: 2127 - protein, 9 aa, synthetic construct
GGLGNDILL

SEQ ID NO: 2128 - protein, 9 aa, synthetic construct
GGGGADVLL

SEQ ID NO: 2129 - protein, 9 aa, synthetic construct
GGIGADTLI

SEQ ID NO: 2130 - protein, 9 aa, synthetic construct
GGVGNDVLN

SEQ ID NO: 2131 - protein, 9 aa, synthetic construct
GGAGRDRLF

SEQ ID NO: 2132 - protein, 9 aa, synthetic construct
GGDGNDTVL

SEQ ID NO: 2133 - protein, 9 aa, synthetic construct
GGAGADTIY

SEQ ID NO: 2134 - protein, 9 aa, synthetic construct
GGAGSDRLY

SEQ ID NO: 2135 - protein, 9 aa, synthetic construct
GGRGNDVLV

SEQ ID NO: 2136 - protein, 9 aa, synthetic construct
GGIGNDTLV

SEQ ID NO: 2137 - protein, 9 aa, synthetic construct
GGNGRDILD

SEQ ID NO: 2138 - protein, 9 aa, synthetic construct
GGTGNDVLL

SEQ ID NO: 2139 - protein, 9 aa, synthetic construct
GGSGADTFT

SEQ ID NO: 2140 - protein, 9 aa, synthetic construct
GGLGNDYLE

SEQ ID NO: 2141 - protein, 9 aa, synthetic construct
GGEGNDTIY

SEQ ID NO: 2142 - protein, 9 aa, synthetic construct
GGDGNDTYV

SEQ ID NO: 2143 - protein, 9 aa, synthetic construct
GGAGDDILH

SEQ ID NO: 2144 - protein, 9 aa, synthetic construct
GGAGTDRLD

SEQ ID NO: 2145 - protein, 9 aa, synthetic construct
GGGGRDTIY

SEQ ID NO: 2146 - protein, 9 aa, synthetic construct
GGAGEDILI

SEQ ID NO: 2147 - protein, 9 aa, synthetic construct
GGRGRDLMD

SEQ ID NO: 2148 - protein, 9 aa, synthetic construct
GGAGLDTLN

SEQ ID NO: 2149 - protein, 9 aa, synthetic construct
GGGGNDSLV

SEQ ID NO: 2150 - protein, 9 aa, synthetic construct
GGDGNDAIN

SEQ ID NO: 2151 - protein, 9 aa, synthetic construct
GGAGDDVFV

SEQ ID NO: 2152 - protein, 9 aa, synthetic construct
GGAGSDTVD

SEQ ID NO: 2153 - protein, 9 aa, synthetic construct
GGAGNDALR

SEQ ID NO: 2154 - protein, 9 aa, synthetic construct
GGAGSDTMT

SEQ ID NO: 2155 - protein, 9 aa, synthetic construct
GGAGADTFL

SEQ ID NO: 2156 - protein, 9 aa, synthetic construct
GGDGDDVLA

SEQ ID NO: 2157 - protein, 9 aa, synthetic construct
GGEGNDALT

SEQ ID NO: 2158 - protein, 9 aa, synthetic construct
GGGGDDVLR

SEQ ID NO: 2159 - protein, 9 aa, synthetic construct
GGGGDDVLT

SEQ ID NO: 2160 - protein, 9 aa, synthetic construct
GGAGDDIYV

SEQ ID NO: 2161 - protein, 9 aa, synthetic construct
GGAGNDEIT

SEQ ID NO: 2162 - protein, 9 aa, synthetic construct
GGAGDDVVS

SEQ ID NO: 2163 - protein, 9 aa, synthetic construct
GGGGDDTLL

SEQ ID NO: 2164 - protein, 9 aa, synthetic construct
GGSGNDTLQ

SEQ ID NO: 2165 - protein, 9 aa, synthetic construct
GGDGADSLD

SEQ ID NO: 2166 - protein, 9 aa, synthetic construct
GGKGNDRLD

SEQ ID NO: 2167 - protein, 9 aa, synthetic construct
GGAGNDRIF

SEQ ID NO: 2168 - protein, 9 aa, synthetic construct
GGTGNDILA

SEQ ID NO: 2169 - protein, 9 aa, synthetic construct
GGAGNDLLK

SEQ ID NO: 2170 - protein, 9 aa, synthetic construct
GGLGNDLID

SEQ ID NO: 2171 - protein, 9 aa, synthetic construct
GGAGKDTLS

SEQ ID NO: 2172 - protein, 9 aa, synthetic construct
GGAGVDKLI

SEQ ID NO: 2173 - protein, 9 aa, synthetic construct
GGGGDDTLV

SEQ ID NO: 2174 - protein, 9 aa, synthetic construct
GGDGNDSLN

SEQ ID NO: 2175 - protein, 9 aa, synthetic construct
GGNGNDSLD

SEQ ID NO: 2176 - protein, 9 aa, synthetic construct
GGGGADRFV

SEQ ID NO: 2177 - protein, 9 aa, synthetic construct
GGQGADTLT

SEQ ID NO: 2178 - protein, 9 aa, synthetic construct
GGKGNDVLM

SEQ ID NO: 2179 - protein, 9 aa, synthetic construct
GGEGSDTLD

SEQ ID NO: 2180 - protein, 9 aa, synthetic construct
GGLGADTFA

SEQ ID NO: 2181 - protein, 9 aa, synthetic construct
GGLGADRLL

SEQ ID NO: 2182 - protein, 9 aa, synthetic construct
GGGGADRLD

SEQ ID NO: 2183 - protein, 9 aa, synthetic construct
GGAGNDLIT

SEQ ID NO: 2184 - protein, 9 aa, synthetic construct
GGAGKDTVR

SEQ ID NO: 2185 - protein, 9 aa, synthetic construct
GGAGDDQIF

SEQ ID NO: 2186 - protein, 9 aa, synthetic construct
GGDGDDTIT

SEQ ID NO: 2187 - protein, 9 aa, synthetic construct
GGAGRDVLI

SEQ ID NO: 2188 - protein, 9 aa, synthetic construct
GGSGDDLFK

SEQ ID NO: 2189 - protein, 9 aa, synthetic construct
GGVGDDYLD

SEQ ID NO: 2190 - protein, 9 aa, synthetic construct
GGEGADIFK

SEQ ID NO: 2191 - protein, 9 aa, synthetic construct
GGEGEDTFV

SEQ ID NO: 2192 - protein, 9 aa, synthetic construct
GGAGRDLLD

SEQ ID NO: 2193 - protein, 9 aa, synthetic construct
GGLGNDSLS

SEQ ID NO: 2194 - protein, 9 aa, synthetic construct
GGDGNDYLT

SEQ ID NO: 2195 - protein, 9 aa, synthetic construct
GGSGDDVLR

SEQ ID NO: 2196 - protein, 9 aa, synthetic construct
GGTGDDRLV

SEQ ID NO: 2197 - protein, 9 aa, synthetic construct
GGGGNDTYV

SEQ ID NO: 2198 - protein, 9 aa, synthetic construct
GGDGDDWID

SEQ ID NO: 2199 - protein, 9 aa, synthetic construct
GGGGADVLT

SEQ ID NO: 2200 - protein, 9 aa, synthetic construct
GGLGADRFV

SEQ ID NO: 2201 - protein, 9 aa, synthetic construct
GGLGADVFV

SEQ ID NO: 2202 - protein, 9 aa, synthetic construct
GGSGADTLY

SEQ ID NO: 2203 - protein, 9 aa, synthetic construct
GGLGDDIYV

SEQ ID NO: 2204 - protein, 9 aa, synthetic construct
GGRGNDTLN

SEQ ID NO: 2205 - protein, 9 aa, synthetic construct
GGLGKDIYR

SEQ ID NO: 2206 - protein, 9 aa, synthetic construct
GGAGTDTLD

SEQ ID NO: 2207 - protein, 9 aa, synthetic construct
GGAGDDFLA

SEQ ID NO: 2208 - protein, 9 aa, synthetic construct
GGEGNDSID

SEQ ID NO: 2209 - protein, 9 aa, synthetic construct
GGSGADTMR

SEQ ID NO: 2210 - protein, 9 aa, synthetic construct
GGGGADTLE

SEQ ID NO: 2211 - protein, 9 aa, synthetic construct
GGVGNDKIY

SEQ ID NO: 2212 - protein, 9 aa, synthetic construct
GGKGDDVLT

SEQ ID NO: 2213 - protein, 9 aa, synthetic construct
GGSGSDVLA

SEQ ID NO: 2214 - protein, 9 aa, synthetic construct
GGAGNDILK

SEQ ID NO: 2215 - protein, 9 aa, synthetic construct
GGRGNDTLL

SEQ ID NO: 2216 - protein, 9 aa, synthetic construct
GGIGNDVLN

SEQ ID NO: 2217 - protein, 9 aa, synthetic construct
GGAGIDRLY

SEQ ID NO: 2218 - protein, 9 aa, synthetic construct
GGIGADRFI

SEQ ID NO: 2219 - protein, 9 aa, synthetic construct
GGLGNDKLY

SEQ ID NO: 2220 - protein, 9 aa, synthetic construct
GGAGADSLA

SEQ ID NO: 2221 - protein, 9 aa, synthetic construct
GGAGDDVIT

SEQ ID NO: 2222 - protein, 9 aa, synthetic construct
GGAGRDSLS

SEQ ID NO: 2223 - protein, 9 aa, synthetic construct
GGAGDDALD

SEQ ID NO: 2224 - protein, 9 aa, synthetic construct
GGAGHDTLE

SEQ ID NO: 2225 - protein, 9 aa, synthetic construct
GGAGNDSLG

SEQ ID NO: 2226 - protein, 9 aa, synthetic construct
GGTGSDTLD

SEQ ID NO: 2227 - protein, 9 aa, synthetic construct
GGTGDDTLA

SEQ ID NO: 2228 - protein, 9 aa, synthetic construct
GGVGNDTLR

SEQ ID NO: 2229 - protein, 9 aa, synthetic construct
GGDGADRLV

SEQ ID NO: 2230 - protein, 9 aa, synthetic construct
GGSGADSFV

SEQ ID NO: 2231 - protein, 9 aa, synthetic construct
GGTGDDVLS

SEQ ID NO: 2232 - protein, 9 aa, synthetic construct
GGDGNDKLD

SEQ ID NO: 2233 - protein, 9 aa, synthetic construct
GGSGGDTLS

SEQ ID NO: 2234 - protein, 9 aa, synthetic construct
GGSGNDVIS

SEQ ID NO: 2235 - protein, 9 aa, synthetic construct
GGVGNDTYI

SEQ ID NO: 2236 - protein, 9 aa, synthetic construct
GGEGRDTIT

SEQ ID NO: 2237 - protein, 9 aa, synthetic construct
GGEGNDTFV

SEQ ID NO: 2238 - protein, 9 aa, synthetic construct
GGAGDDELT

SEQ ID NO: 2239 - protein, 9 aa, synthetic construct
GGQGSDRLQ

SEQ ID NO: 2240 - protein, 9 aa, synthetic construct
GGAGRDTFI

SEQ ID NO: 2241 - protein, 9 aa, synthetic construct
GGLGSDTLN

SEQ ID NO: 2242 - protein, 9 aa, synthetic construct
GGLGKDTLK

SEQ ID NO: 2243 - protein, 9 aa, synthetic construct
GGAGADWFF

SEQ ID NO: 2244 - protein, 9 aa, synthetic construct
GGNGDDVLI

SEQ ID NO: 2245 - protein, 9 aa, synthetic construct
GGRGADLLM

SEQ ID NO: 2246 - protein, 9 aa, synthetic construct
GGNGSDILR

SEQ ID NO: 2247 - protein, 9 aa, synthetic construct
GGDGADTLA

SEQ ID NO: 2248 - protein, 9 aa, synthetic construct
GGLGDDSLD

SEQ ID NO: 2249 - protein, 9 aa, synthetic construct
GGAGNDLMF

SEQ ID NO: 2250 - protein, 9 aa, synthetic construct
GGAGSDLFV

SEQ ID NO: 2251 - protein, 9 aa, synthetic construct
GGEGNDSIL

SEQ ID NO: 2252 - protein, 9 aa, synthetic construct
GGAGGDRLD

SEQ ID NO: 2253 - protein, 9 aa, synthetic construct
GGLGDDLIE

SEQ ID NO: 2254 - protein, 9 aa, synthetic construct
GGAGDDIIV

SEQ ID NO: 2255 - protein, 9 aa, synthetic construct
GGAGSDTFR

SEQ ID NO: 2256 - protein, 9 aa, synthetic construct
GGDGNDWLY

SEQ ID NO: 2257 - protein, 9 aa, synthetic construct
GGAGDDALH

SEQ ID NO: 2258 - protein, 9 aa, synthetic construct
GGDGKDALR

SEQ ID NO: 2259 - protein, 9 aa, synthetic construct
GGTGNDVLF

SEQ ID NO: 2260 - protein, 9 aa, synthetic construct
GGDGNDVLE

SEQ ID NO: 2261 - protein, 9 aa, synthetic construct
GGNGTDTAS

SEQ ID NO: 2262 - protein, 9 aa, synthetic construct
GGAGADSMT

SEQ ID NO: 2263 - protein, 9 aa, synthetic construct
GGGGDDTFV

SEQ ID NO: 2264 - protein, 9 aa, synthetic construct
GGEGADTLT

SEQ ID NO: 2265 - protein, 9 aa, synthetic construct
GGDGNDVIT

SEQ ID NO: 2266 - protein, 9 aa, synthetic construct
GGAGKDRLD

SEQ ID NO: 2267 - protein, 9 aa, synthetic construct
GGAGNDVIR

SEQ ID NO: 2268 - protein, 9 aa, synthetic construct
GGAGADVLR

SEQ ID NO: 2269 - protein, 9 aa, synthetic construct
GGNGNDILY

SEQ ID NO: 2270 - protein, 9 aa, synthetic construct
GGGGADTFR

SEQ ID NO: 2271 - protein, 9 aa, synthetic construct
GGAGRDQVD

SEQ ID NO: 2272 - protein, 9 aa, synthetic construct
GGSGDDQLY

SEQ ID NO: 2273 - protein, 9 aa, synthetic construct
GGGGNDVLV

SEQ ID NO: 2274 - protein, 9 aa, synthetic construct
GGTGFDILN

SEQ ID NO: 2275 - protein, 9 aa, synthetic construct
GGNGNDTLF

SEQ ID NO: 2276 - protein, 9 aa, synthetic construct
GGDGIDKLV

SEQ ID NO: 2277 - protein, 9 aa, synthetic construct
GGSGDDSLS

SEQ ID NO: 2278 - protein, 9 aa, synthetic construct
GGKGDDILD

SEQ ID NO: 2279 - protein, 9 aa, synthetic construct
GGEGNDALS

SEQ ID NO: 2280 - protein, 9 aa, synthetic construct
GGDGDDIIS

SEQ ID NO: 2281 - protein, 9 aa, synthetic construct
GGRGNDTYI

SEQ ID NO: 2282 - protein, 9 aa, synthetic construct
GGEGDDSLF

SEQ ID NO: 2283 - protein, 9 aa, synthetic construct
GGAGNDRIE

SEQ ID NO: 2284 - protein, 9 aa, synthetic construct
GGTGDDTIN

SEQ ID NO: 2285 - protein, 9 aa, synthetic construct
GGEGDDTIY

SEQ ID NO: 2286 - protein, 9 aa, synthetic construct
GGYGDDVLD

SEQ ID NO: 2287 - protein, 9 aa, synthetic construct
GGEGNDGLT

SEQ ID NO: 2288 - protein, 9 aa, synthetic construct
GGEGEDELY

SEQ ID NO: 2289 - protein, 9 aa, synthetic construct
GGSGVDTLA

SEQ ID NO: 2290 - protein, 9 aa, synthetic construct
GGVGDDTYV

SEQ ID NO: 2291 - protein, 9 aa, synthetic construct
GGTGNDSLY

SEQ ID NO: 2292 - protein, 9 aa, synthetic construct
GGDGDDLIV

SEQ ID NO: 2293 - protein, 9 aa, synthetic construct
GGDGDDRIV

SEQ ID NO: 2294 - protein, 9 aa, synthetic construct
GGEGADIIA

SEQ ID NO: 2295 - protein, 9 aa, synthetic construct
GGAGFDTLS

SEQ ID NO: 2296 - protein, 9 aa, synthetic construct
GGAGADVLL

SEQ ID NO: 2297 - protein, 9 aa, synthetic construct
GGTGQDTLN

SEQ ID NO: 2298 - protein, 9 aa, synthetic construct
GGRGNDTLE

SEQ ID NO: 2299 - protein, 9 aa, synthetic construct
GGAGNDDLS

SEQ ID NO: 2300 - protein, 9 aa, synthetic construct
GGNGSDLLI

SEQ ID NO: 2301 - protein, 9 aa, synthetic construct
GGAGADIME

SEQ ID NO: 2302 - protein, 9 aa, synthetic construct
GGLGNDRLN

SEQ ID NO: 2303 - protein, 9 aa, synthetic construct
GGEGNDLLL

SEQ ID NO: 2304 - protein, 9 aa, synthetic construct
GGSGDDVLF

SEQ ID NO: 2305 - protein, 9 aa, synthetic construct
GGLGRDTLT

SEQ ID NO: 2306 - protein, 9 aa, synthetic construct
GGAGADQLY

SEQ ID NO: 2307 - protein, 9 aa, synthetic construct
GGDGADSLY

SEQ ID NO: 2308 - protein, 9 aa, synthetic construct
GGLGTDTLI

SEQ ID NO: 2309 - protein, 9 aa, synthetic construct
GGAGNDALL

SEQ ID NO: 2310 - protein, 9 aa, synthetic construct
GGAGSDTFA

SEQ ID NO: 2311 - protein, 9 aa, synthetic construct
GGKGNDSLT

SEQ ID NO: 2312 - protein, 9 aa, synthetic construct
GGAGADLLR

SEQ ID NO: 2313 - protein, 9 aa, synthetic construct
GGLGADTLE

SEQ ID NO: 2314 - protein, 9 aa, synthetic construct
GGVGNDVFV

SEQ ID NO: 2315 - protein, 9 aa, synthetic construct
GGRGADTLI

SEQ ID NO: 2316 - protein, 9 aa, synthetic construct
GGAGDDFVN

SEQ ID NO: 2317 - protein, 9 aa, synthetic construct
GGGGNDRLN

SEQ ID NO: 2318 - protein, 9 aa, synthetic construct
GGDGADTLF

SEQ ID NO: 2319 - protein, 9 aa, synthetic construct
GGEGDDVLH

SEQ ID NO: 2320 - protein, 9 aa, synthetic construct
GGDGADVLN

SEQ ID NO: 2321 - protein, 9 aa, synthetic construct
GGSGGDTLT

SEQ ID NO: 2322 - protein, 9 aa, synthetic construct
GGTGADTFI

SEQ ID NO: 2323 - protein, 9 aa, synthetic construct
GGAGKDVLS

SEQ ID NO: 2324 - protein, 9 aa, synthetic construct
GGLGNDILS

SEQ ID NO: 2325 - protein, 9 aa, synthetic construct
GGDGNDTFL

SEQ ID NO: 2326 - protein, 9 aa, synthetic construct
GGIGNDVLD

SEQ ID NO: 2327 - protein, 9 aa, synthetic construct
GGNGDDSLD

SEQ ID NO: 2328 - protein, 9 aa, synthetic construct
GGGGNDTIY

SEQ ID NO: 2329 - protein, 9 aa, synthetic construct
GGSGDDQLD

SEQ ID NO: 2330 - protein, 9 aa, synthetic construct
GGLGSDILM

SEQ ID NO: 2331 - protein, 9 aa, synthetic construct
GGEGDDVLV

SEQ ID NO: 2332 - protein, 9 aa, synthetic construct
GGEGDDLLV

SEQ ID NO: 2333 - protein, 9 aa, synthetic construct
GGAGDDYLE

SEQ ID NO: 2334 - protein, 9 aa, synthetic construct
GGAGADALS

SEQ ID NO: 2335 - protein, 9 aa, synthetic construct
GGGGNDVLL

SEQ ID NO: 2336 - protein, 9 aa, synthetic construct
GGLGDDTID

SEQ ID NO: 2337 - protein, 9 aa, synthetic construct
GGDGNDTVS

SEQ ID NO: 2338 - protein, 9 aa, synthetic construct
GGTGADTLA

SEQ ID NO: 2339 - protein, 9 aa, synthetic construct
GGWGNDKLN

SEQ ID NO: 2340 - protein, 9 aa, synthetic construct
GGDGNDYID

SEQ ID NO: 2341 - protein, 9 aa, synthetic construct
GGNGADTLS

SEQ ID NO: 2342 - protein, 9 aa, synthetic construct
GGSGNDTIF

SEQ ID NO: 2343 - protein, 9 aa, synthetic construct
GGLGNDSYV

SEQ ID NO: 2344 - protein, 9 aa, synthetic construct
GGAGNDLIN

SEQ ID NO: 2345 - protein, 9 aa, synthetic construct
GGGGNDVLY

SEQ ID NO: 2346 - protein, 9 aa, synthetic construct
GGAGDDSLE

SEQ ID NO: 2347 - protein, 9 aa, synthetic construct
GGDGNDTIA

SEQ ID NO: 2348 - protein, 9 aa, synthetic construct
GGAGADALT

SEQ ID NO: 2349 - protein, 9 aa, synthetic construct
GGDGNDVIF

SEQ ID NO: 2350 - protein, 9 aa, synthetic construct
GGLGADDLT

SEQ ID NO: 2351 - protein, 9 aa, synthetic construct
GGAGNDWLY

SEQ ID NO: 2352 - protein, 9 aa, synthetic construct
GGAGDDIMF

SEQ ID NO: 2353 - protein, 9 aa, synthetic construct
GGAGDDRIE

SEQ ID NO: 2354 - protein, 9 aa, synthetic construct
GGKGNDTYG

SEQ ID NO: 2355 - protein, 9 aa, synthetic construct
GGAGDDKID

SEQ ID NO: 2356 - protein, 9 aa, synthetic construct
GGEGDDYLD

SEQ ID NO: 2357 - protein, 9 aa, synthetic construct
GGAGNDYLI

SEQ ID NO: 2358 - protein, 9 aa, synthetic construct
GGSGNDTMT

SEQ ID NO: 2359 - protein, 9 aa, synthetic construct
GGEGSDTID

SEQ ID NO: 2360 - protein, 9 aa, synthetic construct
GGTGNDYLD

SEQ ID NO: 2361 - protein, 9 aa, synthetic construct
GGAGKDSLY

SEQ ID NO: 2362 - protein, 9 aa, synthetic construct
GGEGNDTYL

SEQ ID NO: 2363 - protein, 9 aa, synthetic construct
GGRGNDILF

SEQ ID NO: 2364 - protein, 9 aa, synthetic construct
GGAGADALY

SEQ ID NO: 2365 - protein, 9 aa, synthetic construct
GGAGSDIFV

SEQ ID NO: 2366 - protein, 9 aa, synthetic construct
GGDGSDILI

SEQ ID NO: 2367 - protein, 9 aa, synthetic construct
GGLGVDTLT

SEQ ID NO: 2368 - protein, 9 aa, synthetic construct
GGDGNDIIF

SEQ ID NO: 2369 - protein, 9 aa, synthetic construct
GGEGDDVLF

SEQ ID NO: 2370 - protein, 9 aa, synthetic construct
GGGGDDTIY

SEQ ID NO: 2371 - protein, 9 aa, synthetic construct
GGSGDDLLY

SEQ ID NO: 2372 - protein, 9 aa, synthetic construct
GGEGDDSIS

SEQ ID NO: 2373 - protein, 9 aa, synthetic construct
GGAGFDTLD

SEQ ID NO: 2374 - protein, 9 aa, synthetic construct
GGQGNDDLA

SEQ ID NO: 2375 - protein, 9 aa, synthetic construct
GGTGNDSID

SEQ ID NO: 2376 - protein, 9 aa, synthetic construct
GGDGNDGLR

SEQ ID NO: 2377 - protein, 9 aa, synthetic construct
GGDGTDLLA

SEQ ID NO: 2378 - protein, 9 aa, synthetic construct
GGSGDDTLE

SEQ ID NO: 2379 - protein, 9 aa, synthetic construct
GGEGSDTLI

SEQ ID NO: 2380 - protein, 9 aa, synthetic construct
GGNGSDTLI

SEQ ID NO: 2381 - protein, 9 aa, synthetic construct
GGAGDDTVL

SEQ ID NO: 2382 - protein, 9 aa, synthetic construct
GGGGNDRLS

SEQ ID NO: 2383 - protein, 9 aa, synthetic construct
GGGGRDTFV

SEQ ID NO: 2384 - protein, 9 aa, synthetic construct
GGGGNDTLQ

SEQ ID NO: 2385 - protein, 9 aa, synthetic construct
GGEGDDTLS

SEQ ID NO: 2386 - protein, 9 aa, synthetic construct
GGTGSDKLD

SEQ ID NO: 2387 - protein, 9 aa, synthetic construct
GGQGADTID

SEQ ID NO: 2388 - protein, 9 aa, synthetic construct
GGAGSDELY

SEQ ID NO: 2389 - protein, 9 aa, synthetic construct
GGSGNDALF

SEQ ID NO: 2390 - protein, 9 aa, synthetic construct
GGAGSDILV

SEQ ID NO: 2391 - protein, 9 aa, synthetic construct
GGTGDDTLR

SEQ ID NO: 2392 - protein, 9 aa, synthetic construct
GGDGSDSLD

SEQ ID NO: 2393 - protein, 9 aa, synthetic construct
GGVGTDTLI

SEQ ID NO: 2394 - protein, 9 aa, synthetic construct
GGAGDDLIY

SEQ ID NO: 2395 - protein, 9 aa, synthetic construct
GGAGVDTVV

SEQ ID NO: 2396 - protein, 9 aa, synthetic construct
GGDGSDTLD

SEQ ID NO: 2397 - protein, 9 aa, synthetic construct
GGDGSDTLA

SEQ ID NO: 2398 - protein, 9 aa, synthetic construct
GGEGNDTIT

SEQ ID NO: 2399 - protein, 9 aa, synthetic construct
GGTGADTIT

SEQ ID NO: 2400 - protein, 9 aa, synthetic construct
GGSGNDVFV

SEQ ID NO: 2401 - protein, 9 aa, synthetic construct
GGAGSDSLD

SEQ ID NO: 2402 - protein, 9 aa, synthetic construct
GGAGNDTYF

SEQ ID NO: 2403 - protein, 9 aa, synthetic construct
GGKGADTLL

SEQ ID NO: 2404 - protein, 9 aa, synthetic construct
GGSGNDQLD

SEQ ID NO: 2405 - protein, 9 aa, synthetic construct
GGSGNDKLT

SEQ ID NO: 2406 - protein, 9 aa, synthetic construct
GGDGADTIL

SEQ ID NO: 2407 - protein, 9 aa, synthetic construct
GGGGADTIT

SEQ ID NO: 2408 - protein, 9 aa, synthetic construct
GGGGADVLI

SEQ ID NO: 2409 - protein, 9 aa, synthetic construct
GGDGADIFV

SEQ ID NO: 2410 - protein, 9 aa, synthetic construct
GGAGGDTLL

SEQ ID NO: 2411 - protein, 9 aa, synthetic construct
GGTGRDTLD

SEQ ID NO: 2412 - protein, 9 aa, synthetic construct
GGAGIDTVD

SEQ ID NO: 2413 - protein, 9 aa, synthetic construct
GGGGNDLID

SEQ ID NO: 2414 - protein, 9 aa, synthetic construct
GGAGIDTLD

SEQ ID NO: 2415 - protein, 9 aa, synthetic construct
GGDGDDIIY

SEQ ID NO: 2416 - protein, 9 aa, synthetic construct
GGAGADELW

SEQ ID NO: 2417 - protein, 9 aa, synthetic construct
GGNGDDYLD

SEQ ID NO: 2418 - protein, 9 aa, synthetic construct
GGNGNDRLS

SEQ ID NO: 2419 - protein, 9 aa, synthetic construct
GGDGADSLL

SEQ ID NO: 2420 - protein, 9 aa, synthetic construct
GGDGDDKLT

SEQ ID NO: 2421 - protein, 9 aa, synthetic construct
GGAGRDRLS

SEQ ID NO: 2422 - protein, 9 aa, synthetic construct
GGDGDDRLT

SEQ ID NO: 2423 - protein, 9 aa, synthetic construct
GGDGADKLF

SEQ ID NO: 2424 - protein, 9 aa, synthetic construct
GGTGADRLI

SEQ ID NO: 2425 - protein, 9 aa, synthetic construct
GGDGDDTLH

SEQ ID NO: 2426 - protein, 9 aa, synthetic construct
GGRGNDVLI

SEQ ID NO: 2427 - protein, 9 aa, synthetic construct
GGKGNDLLS

SEQ ID NO: 2428 - protein, 9 aa, synthetic construct
GGDGSDIFK

SEQ ID NO: 2429 - protein, 9 aa, synthetic construct
GGLGDDTLA

SEQ ID NO: 2430 - protein, 9 aa, synthetic construct
GGTGADSLV

SEQ ID NO: 2431 - protein, 9 aa, synthetic construct
GGGGDDWIF

SEQ ID NO: 2432 - protein, 9 aa, synthetic construct
GGAGDDSLG

SEQ ID NO: 2433 - protein, 9 aa, synthetic construct
GGLGQDTMT

SEQ ID NO: 2434 - protein, 9 aa, synthetic construct
GGLGHDTLT

SEQ ID NO: 2435 - protein, 9 aa, synthetic construct
GGTGADKLY

SEQ ID NO: 2436 - protein, 9 aa, synthetic construct
GGAGNDLVD

SEQ ID NO: 2437 - protein, 9 aa, synthetic construct
GGFGNDTLD

SEQ ID NO: 2438 - protein, 9 aa, synthetic construct
GGGGNDVID

SEQ ID NO: 2439 - protein, 9 aa, synthetic construct
GGEGDDRLE

SEQ ID NO: 2440 - protein, 9 aa, synthetic construct
GGTGADSMT

SEQ ID NO: 2441 - protein, 9 aa, synthetic construct
GGDGNDRIY

SEQ ID NO: 2442 - protein, 9 aa, synthetic construct
GGSGDDTIL

SEQ ID NO: 2443 - protein, 9 aa, synthetic construct
GGLGDDTLY

SEQ ID NO: 2444 - protein, 9 aa, synthetic construct
GGNGNDRLE

SEQ ID NO: 2445 - protein, 9 aa, synthetic construct
GGWGNDRLY

SEQ ID NO: 2446 - protein, 9 aa, synthetic construct
GGKGADILT

SEQ ID NO: 2447 - protein, 9 aa, synthetic construct
GGAGSDRLE

SEQ ID NO: 2448 - protein, 9 aa, synthetic construct
GGDGDDWLF

SEQ ID NO: 2449 - protein, 9 aa, synthetic construct
GGAGDDSMD

SEQ ID NO: 2450 - protein, 9 aa, synthetic construct
GGAGADILR

SEQ ID NO: 2451 - protein, 9 aa, synthetic construct
GGAGHDTLL

SEQ ID NO: 2452 - protein, 9 aa, synthetic construct
GGAGNDRAY

SEQ ID NO: 2453 - protein, 9 aa, synthetic construct
GGAGADRFY

SEQ ID NO: 2454 - protein, 9 aa, synthetic construct
GGLGDDTYF

SEQ ID NO: 2455 - protein, 9 aa, synthetic construct
GGVGDDTLD

SEQ ID NO: 2456 - protein, 9 aa, synthetic construct
GGNGNDTLK

SEQ ID NO: 2457 - protein, 9 aa, synthetic construct
GGAGSDSYV

SEQ ID NO: 2458 - protein, 9 aa, synthetic construct
GGPGRDTLD

SEQ ID NO: 2459 - protein, 9 aa, synthetic construct
GGDGNDLLQ

SEQ ID NO: 2460 - protein, 9 aa, synthetic construct
GGAGSDRLD

SEQ ID NO: 2461 - protein, 9 aa, synthetic construct
GGIGADTLS

SEQ ID NO: 2462 - protein, 9 aa, synthetic construct
GGAGGDQLF

SEQ ID NO: 2463 - protein, 9 aa, synthetic construct
GGGGQDTID

SEQ ID NO: 2464 - protein, 9 aa, synthetic construct
GGVGADTLM

SEQ ID NO: 2465 - protein, 9 aa, synthetic construct
GGNGNDLAN

SEQ ID NO: 2466 - protein, 9 aa, synthetic construct
GGAGNDALA

SEQ ID NO: 2467 - protein, 9 aa, synthetic construct
GGDGNDLID

SEQ ID NO: 2468 - protein, 9 aa, synthetic construct
GGSGTDTAV

SEQ ID NO: 2469 - protein, 9 aa, synthetic construct
GGAGRDTLY

SEQ ID NO: 2470 - protein, 9 aa, synthetic construct
GGGGNDLLR

SEQ ID NO: 2471 - protein, 9 aa, synthetic construct
GGDGNDSLA

SEQ ID NO: 2472 - protein, 9 aa, synthetic construct
GGGGNDLLE

SEQ ID NO: 2473 - protein, 9 aa, synthetic construct
GGDGNDELF

SEQ ID NO: 2474 - protein, 9 aa, synthetic construct
GGAGNDELI

SEQ ID NO: 2475 - protein, 9 aa, synthetic construct
GGKGNDTLL

SEQ ID NO: 2476 - protein, 9 aa, synthetic construct
GGPGNDTLN

SEQ ID NO: 2477 - protein, 9 aa, synthetic construct
GGGGNDLLS

SEQ ID NO: 2478 - protein, 9 aa, synthetic construct
GGQGDDTLL

SEQ ID NO: 2479 - protein, 9 aa, synthetic construct
GGDGDDRLI

SEQ ID NO: 2480 - protein, 9 aa, synthetic construct
GGAGQDSLF

SEQ ID NO: 2481 - protein, 9 aa, synthetic construct
GGTGADSLI

SEQ ID NO: 2482 - protein, 9 aa, synthetic construct
GGDGNDLLA

SEQ ID NO: 2483 - protein, 9 aa, synthetic construct
GGVGADTFV

SEQ ID NO: 2484 - protein, 9 aa, synthetic construct
GGAGNDFLS

SEQ ID NO: 2485 - protein, 9 aa, synthetic construct
GGAGRDLLI

SEQ ID NO: 2486 - protein, 9 aa, synthetic construct
GGNGNDVLV

SEQ ID NO: 2487 - protein, 9 aa, synthetic construct
GGNGDDTLE

SEQ ID NO: 2488 - protein, 9 aa, synthetic construct
GGAGGDTLN

SEQ ID NO: 2489 - protein, 9 aa, synthetic construct
GGAGNDFLR

SEQ ID NO: 2490 - protein, 9 aa, synthetic construct
GGGGDDILV

SEQ ID NO: 2491 - protein, 9 aa, synthetic construct
GGGGDDILT

SEQ ID NO: 2492 - protein, 9 aa, synthetic construct
GGSGDDILT

SEQ ID NO: 2493 - protein, 9 aa, synthetic construct
GGGGGDTLR

SEQ ID NO: 2494 - protein, 9 aa, synthetic construct
GGAGVDTVS

SEQ ID NO: 2495 - protein, 9 aa, synthetic construct
GGAGADVIN

SEQ ID NO: 2496 - protein, 9 aa, synthetic construct
GGDGDDVII

SEQ ID NO: 2497 - protein, 9 aa, synthetic construct
GGAGNDVIF

SEQ ID NO: 2498 - protein, 9 aa, synthetic construct
GGGGADKLY

SEQ ID NO: 2499 - protein, 9 aa, synthetic construct
GGRGADELQ

SEQ ID NO: 2500 - protein, 9 aa, synthetic construct
GGNGKDDLN

SEQ ID NO: 2501 - protein, 9 aa, synthetic construct
GGNGNDILR

SEQ ID NO: 2502 - protein, 9 aa, synthetic construct
GGFGADSIT

SEQ ID NO: 2503 - protein, 9 aa, synthetic construct
GGSGSDTLY

SEQ ID NO: 2504 - protein, 9 aa, synthetic construct
GGGGDDRLF

SEQ ID NO: 2505 - protein, 9 aa, synthetic construct
GGAGADMLI

SEQ ID NO: 2506 - protein, 9 aa, synthetic construct
GGDGNDFIN

SEQ ID NO: 2507 - protein, 9 aa, synthetic construct
GGAGDDRLQ

SEQ ID NO: 2508 - protein, 9 aa, synthetic construct
GGSGNDELS

SEQ ID NO: 2509 - protein, 9 aa, synthetic construct
GGSGDDTYV

SEQ ID NO: 2510 - protein, 9 aa, synthetic construct
GGDGADTIS

SEQ ID NO: 2511 - protein, 9 aa, synthetic construct
GGVGNDFLE

SEQ ID NO: 2512 - protein, 9 aa, synthetic construct
GGPGADTLT

SEQ ID NO: 2513 - protein, 9 aa, synthetic construct
GGDGDDTYY

SEQ ID NO: 2514 - protein, 9 aa, synthetic construct
GGKGDDTLE

SEQ ID NO: 2515 - protein, 9 aa, synthetic construct
GGSGNDTFI

SEQ ID NO: 2516 - protein, 9 aa, synthetic construct
GGNGDDTLS

SEQ ID NO: 2517 - protein, 9 aa, synthetic construct
GGRGADKLR

SEQ ID NO: 2518 - protein, 9 aa, synthetic construct
GGAGADVLE

SEQ ID NO: 2519 - protein, 9 aa, synthetic construct
GGAGADVIY

SEQ ID NO: 2520 - protein, 9 aa, synthetic construct
GGDGDDRLA

SEQ ID NO: 2521 - protein, 9 aa, synthetic construct
GGAGDDEIH

SEQ ID NO: 2522 - protein, 9 aa, synthetic construct
GGEGADRMS

SEQ ID NO: 2523 - protein, 9 aa, synthetic construct
GGSGNDNLQ

SEQ ID NO: 2524 - protein, 9 aa, synthetic construct
GGAGADVIT

SEQ ID NO: 2525 - protein, 9 aa, synthetic construct
GGAGSDVII

SEQ ID NO: 2526 - protein, 9 aa, synthetic construct
GGTGNDIYY

SEQ ID NO: 2527 - protein, 9 aa, synthetic construct
GGEGSDTYR

SEQ ID NO: 2528 - protein, 9 aa, synthetic construct
GGAGNDQIS

SEQ ID NO: 2529 - protein, 9 aa, synthetic construct
GGDGSDTLV

SEQ ID NO: 2530 - protein, 9 aa, synthetic construct
GGEGRDDVN

SEQ ID NO: 2531 - protein, 9 aa, synthetic construct
GGRGDDTYI

SEQ ID NO: 2532 - protein, 9 aa, synthetic construct
GGSGADSLD

SEQ ID NO: 2533 - protein, 9 aa, synthetic construct
GGSGNDLLT

SEQ ID NO: 2534 - protein, 9 aa, synthetic construct
GGSGADSIT

SEQ ID NO: 2535 - protein, 9 aa, synthetic construct
GGDGNDSIT

SEQ ID NO: 2536 - protein, 9 aa, synthetic construct
GGAGHDRLA

SEQ ID NO: 2537 - protein, 9 aa, synthetic construct
GGDGADRLE

SEQ ID NO: 2538 - protein, 9 aa, synthetic construct
GGAGDDVIE

SEQ ID NO: 2539 - protein, 9 aa, synthetic construct
GGTGADRLV

SEQ ID NO: 2540 - protein, 9 aa, synthetic construct
GGSGNDSLN

SEQ ID NO: 2541 - protein, 9 aa, synthetic construct
GGIGSDTYV

SEQ ID NO: 2542 - protein, 9 aa, synthetic construct
GGAGADNFE

SEQ ID NO: 2543 - protein, 9 aa, synthetic construct
GGGGDDLLD

SEQ ID NO: 2544 - protein, 9 aa, synthetic construct
GGGGNDRLT

SEQ ID NO: 2545 - protein, 9 aa, synthetic construct
GGLGADVLR

SEQ ID NO: 2546 - protein, 9 aa, synthetic construct
GGSGNDQLN

SEQ ID NO: 2547 - protein, 9 aa, synthetic construct
GGAGADLLV

SEQ ID NO: 2548 - protein, 9 aa, synthetic construct
GGEGADLMV

SEQ ID NO: 2549 - protein, 9 aa, synthetic construct
GGTGNDQLI

SEQ ID NO: 2550 - protein, 9 aa, synthetic construct
GGDGDDFLN

SEQ ID NO: 2551 - protein, 9 aa, synthetic construct
GGAGQDYMN

SEQ ID NO: 2552 - protein, 9 aa, synthetic construct
GGFGDDSIL

SEQ ID NO: 2553 - protein, 9 aa, synthetic construct
GGGGDDILM

SEQ ID NO: 2554 - protein, 9 aa, synthetic construct
GGNGDDTLL

SEQ ID NO: 2555 - protein, 9 aa, synthetic construct
GGSGNDRIY

SEQ ID NO: 2556 - protein, 9 aa, synthetic construct
GGDGDDELR

SEQ ID NO: 2557 - protein, 9 aa, synthetic construct
GGKGNDTFY

SEQ ID NO: 2558 - protein, 9 aa, synthetic construct
GGAGSDILD

SEQ ID NO: 2559 - protein, 9 aa, synthetic construct
GGDGDDYLA

SEQ ID NO: 2560 - protein, 9 aa, synthetic construct
GGSGNDRFV

SEQ ID NO: 2561 - protein, 9 aa, synthetic construct
GGAGADMLD

SEQ ID NO: 2562 - protein, 9 aa, synthetic construct
GGDGNDTIV

SEQ ID NO: 2563 - protein, 9 aa, synthetic construct
GGDGSDTLS

SEQ ID NO: 2564 - protein, 9 aa, synthetic construct
GGAGADQLL

SEQ ID NO: 2565 - protein, 9 aa, synthetic construct
GGDGDDTYV

SEQ ID NO: 2566 - protein, 9 aa, synthetic construct
GGSGTDTLT

SEQ ID NO: 2567 - protein, 9 aa, synthetic construct
GGTGNDSIS

SEQ ID NO: 2568 - protein, 9 aa, synthetic construct
GGDGADTLE

SEQ ID NO: 2569 - protein, 9 aa, synthetic construct
GGEGNDRLY

SEQ ID NO: 2570 - protein, 9 aa, synthetic construct
GGNGADTLI

SEQ ID NO: 2571 - protein, 9 aa, synthetic construct
GGEGADLFR

SEQ ID NO: 2572 - protein, 9 aa, synthetic construct
GGAGNDYID

SEQ ID NO: 2573 - protein, 9 aa, synthetic construct
GGDGDDIIR

SEQ ID NO: 2574 - protein, 9 aa, synthetic construct
GGGGNDYLD

SEQ ID NO: 2575 - protein, 9 aa, synthetic construct
GGAGRDRID

SEQ ID NO: 2576 - protein, 9 aa, synthetic construct
GGAGVDRLY

SEQ ID NO: 2577 - protein, 9 aa, synthetic construct
GGSGADVLN

SEQ ID NO: 2578 - protein, 9 aa, synthetic construct
GGLGNDQLY

SEQ ID NO: 2579 - protein, 9 aa, synthetic construct
GGTGNDSLN

SEQ ID NO: 2580 - protein, 9 aa, synthetic construct
GGSGNDVMQ

SEQ ID NO: 2581 - protein, 9 aa, synthetic construct
GGSGADILN

SEQ ID NO: 2582 - protein, 9 aa, synthetic construct
GGDGRDTLS

SEQ ID NO: 2583 - protein, 9 aa, synthetic construct
GGNGDDEIY

SEQ ID NO: 2584 - protein, 9 aa, synthetic construct
GGSGADVLL

SEQ ID NO: 2585 - protein, 9 aa, synthetic construct
GGDGQDTIT

SEQ ID NO: 2586 - protein, 9 aa, synthetic construct
GGSGADTFM

SEQ ID NO: 2587 - protein, 9 aa, synthetic construct
GGEGDDLLT

SEQ ID NO: 2588 - protein, 9 aa, synthetic construct
GGSGADKLY

SEQ ID NO: 2589 - protein, 9 aa, synthetic construct
GGSGADTID

SEQ ID NO: 2590 - protein, 9 aa, synthetic construct
GGTGDDTLV

SEQ ID NO: 2591 - protein, 9 aa, synthetic construct
GGAGNDTMN

SEQ ID NO: 2592 - protein, 9 aa, synthetic construct
GGVGNDYLS

SEQ ID NO: 2593 - protein, 9 aa, synthetic construct
GGGGDDLLL

SEQ ID NO: 2594 - protein, 9 aa, synthetic construct
GGAGADTMN

SEQ ID NO: 2595 - protein, 9 aa, synthetic construct
GGAGNDTYT

SEQ ID NO: 2596 - protein, 9 aa, synthetic construct
GGEGNDTLA

SEQ ID NO: 2597 - protein, 9 aa, synthetic construct
GGAGFDEAS

SEQ ID NO: 2598 - protein, 9 aa, synthetic construct
GGAGDDALI

SEQ ID NO: 2599 - protein, 9 aa, synthetic construct
GGAGTDVII

SEQ ID NO: 2600 - protein, 9 aa, synthetic construct
GGAGDDALL

SEQ ID NO: 2601 - protein, 9 aa, synthetic construct
GGDGNDLIY

SEQ ID NO: 2602 - protein, 9 aa, synthetic construct
GGLGDDSLV

SEQ ID NO: 2603 - protein, 9 aa, synthetic construct
GGEGDDSLL

SEQ ID NO: 2604 - protein, 9 aa, synthetic construct
GGAGNDKLS

SEQ ID NO: 2605 - protein, 9 aa, synthetic construct
GGNGADTFI

SEQ ID NO: 2606 - protein, 9 aa, synthetic construct
GGAGDDALN

SEQ ID NO: 2607 - protein, 9 aa, synthetic construct
GGKGNDILS

SEQ ID NO: 2608 - protein, 9 aa, synthetic construct
GGTGDDILN

SEQ ID NO: 2609 - protein, 9 aa, synthetic construct
GGAGNDTVY

SEQ ID NO: 2610 - protein, 9 aa, synthetic construct
GGDGNDRIT

SEQ ID NO: 2611 - protein, 9 aa, synthetic construct
GGAGDDLLK

SEQ ID NO: 2612 - protein, 9 aa, synthetic construct
GGEGDDQLF

SEQ ID NO: 2613 - protein, 9 aa, synthetic construct
GGDGSDTLY

SEQ ID NO: 2614 - protein, 9 aa, synthetic construct
GGEGDDWLF

SEQ ID NO: 2615 - protein, 9 aa, synthetic construct
GGAGDDALA

SEQ ID NO: 2616 - protein, 9 aa, synthetic construct
GGSGDDVLN

SEQ ID NO: 2617 - protein, 9 aa, synthetic construct
GGAGNDLMQ

SEQ ID NO: 2618 - protein, 9 aa, synthetic construct
GGAGHDSLF

SEQ ID NO: 2619 - protein, 9 aa, synthetic construct
GGAGNDVIL

SEQ ID NO: 2620 - protein, 9 aa, synthetic construct
GGAGDDTLW

SEQ ID NO: 2621 - protein, 9 aa, synthetic construct
GGTGKDVFS

SEQ ID NO: 2622 - protein, 9 aa, synthetic construct
GGDGNDTLW

SEQ ID NO: 2623 - protein, 9 aa, synthetic construct
GGRGSDVFV

SEQ ID NO: 2624 - protein, 9 aa, synthetic construct
GGAGSDLLV

SEQ ID NO: 2625 - protein, 9 aa, synthetic construct
GGNGDDILE

SEQ ID NO: 2626 - protein, 9 aa, synthetic construct
GGTGNDILL

SEQ ID NO: 2627 - protein, 9 aa, synthetic construct
GGVGADRFV

SEQ ID NO: 2628 - protein, 9 aa, synthetic construct
GGAGHDILS

SEQ ID NO: 2629 - protein, 9 aa, synthetic construct
GGAGIDTLR

SEQ ID NO: 2630 - protein, 9 aa, synthetic construct
GGKGDDVLS

SEQ ID NO: 2631 - protein, 9 aa, synthetic construct
GGIGGDTIS

SEQ ID NO: 2632 - protein, 9 aa, synthetic construct
GGAGNDLIF

SEQ ID NO: 2633 - protein, 9 aa, synthetic construct
GGQGNDRLS

SEQ ID NO: 2634 - protein, 9 aa, synthetic construct
GGGGDDTLA

SEQ ID NO: 2635 - protein, 9 aa, synthetic construct
GGSGDDRFT

SEQ ID NO: 2636 - protein, 9 aa, synthetic construct
GGAGNDRLG

SEQ ID NO: 2637 - protein, 9 aa, synthetic construct
GGDGIDYLH

SEQ ID NO: 2638 - protein, 9 aa, synthetic construct
GGQGDDTLS

SEQ ID NO: 2639 - protein, 9 aa, synthetic construct
GGEGNDKLY

SEQ ID NO: 2640 - protein, 9 aa, synthetic construct
GGPGDDTID

SEQ ID NO: 2641 - protein, 9 aa, synthetic construct
GGTGADVLD

SEQ ID NO: 2642 - protein, 9 aa, synthetic construct
GGAGDDELR

SEQ ID NO: 2643 - protein, 9 aa, synthetic construct
GGNGNDLLN

SEQ ID NO: 2644 - protein, 9 aa, synthetic construct
GGDGFDFLD

SEQ ID NO: 2645 - protein, 9 aa, synthetic construct
GGIGNDRLI

SEQ ID NO: 2646 - protein, 9 aa, synthetic construct
GGAGRDAFV

SEQ ID NO: 2647 - protein, 9 aa, synthetic construct
GGAGTDNLS

SEQ ID NO: 2648 - protein, 9 aa, synthetic construct
GGAGDDDLF

SEQ ID NO: 2649 - protein, 9 aa, synthetic construct
GGAGNDMLF

SEQ ID NO: 2650 - protein, 9 aa, synthetic construct
GGDGADRLI

SEQ ID NO: 2651 - protein, 9 aa, synthetic construct
GGAGSDTFI

SEQ ID NO: 2652 - protein, 9 aa, synthetic construct
GGTGNDTLQ

SEQ ID NO: 2653 - protein, 9 aa, synthetic construct
GGTGADTLR

SEQ ID NO: 2654 - protein, 9 aa, synthetic construct
GGSGDDLLV

SEQ ID NO: 2655 - protein, 9 aa, synthetic construct
GGIGNDRLY

SEQ ID NO: 2656 - protein, 9 aa, synthetic construct
GGIGNDTIY

SEQ ID NO: 2657 - protein, 9 aa, synthetic construct
GGTGADTMA

SEQ ID NO: 2658 - protein, 9 aa, synthetic construct
GGAGNDRMS

SEQ ID NO: 2659 - protein, 9 aa, synthetic construct
GGLGNDTLE

SEQ ID NO: 2660 - protein, 9 aa, synthetic construct
GGNGNDTID

SEQ ID NO: 2661 - protein, 9 aa, synthetic construct
GGAGQDTMT

SEQ ID NO: 2662 - protein, 9 aa, synthetic construct
GGSGSDILT

SEQ ID NO: 2663 - protein, 9 aa, synthetic construct
GGDGHDHLD

SEQ ID NO: 2664 - protein, 9 aa, synthetic construct
GGSGNDDLS

SEQ ID NO: 2665 - protein, 9 aa, synthetic construct
GGSGSDTLV

SEQ ID NO: 2666 - protein, 9 aa, synthetic construct
GGSGDDQLF

SEQ ID NO: 2667 - protein, 9 aa, synthetic construct
GGGGNDNLH

SEQ ID NO: 2668 - protein, 9 aa, synthetic construct
GGVGNDTID

SEQ ID NO: 2669 - protein, 9 aa, synthetic construct
GGAGDDYLQ

SEQ ID NO: 2670 - protein, 9 aa, synthetic construct
GGSGDDILS

SEQ ID NO: 2671 - protein, 9 aa, synthetic construct
GGIGNDSLY

SEQ ID NO: 2672 - protein, 9 aa, synthetic construct
GGLGADLLD

SEQ ID NO: 2673 - protein, 9 aa, synthetic construct
GGAGADALN

SEQ ID NO: 2674 - protein, 9 aa, synthetic construct
GGMGNDTLN

SEQ ID NO: 2675 - protein, 9 aa, synthetic construct
GGGGADIFD

SEQ ID NO: 2676 - protein, 9 aa, synthetic construct
GGAGDDDLY

SEQ ID NO: 2677 - protein, 9 aa, synthetic construct
GGLGADRLE

SEQ ID NO: 2678 - protein, 9 aa, synthetic construct
GGAGADSLE

SEQ ID NO: 2679 - protein, 9 aa, synthetic construct
GGKGDDIMT

SEQ ID NO: 2680 - protein, 9 aa, synthetic construct
GGQGDDVLD

SEQ ID NO: 2681 - protein, 9 aa, synthetic construct
GGNGRDTLI

SEQ ID NO: 2682 - protein, 9 aa, synthetic construct
GGDGSDSVD

SEQ ID NO: 2683 - protein, 9 aa, synthetic construct
GGAGDDYID

SEQ ID NO: 2684 - protein, 9 aa, synthetic construct
GGLGADTIS

SEQ ID NO: 2685 - protein, 9 aa, synthetic construct
GGDGADTFQ

SEQ ID NO: 2686 - protein, 9 aa, synthetic construct
GGSGNDFLD

SEQ ID NO: 2687 - protein, 9 aa, synthetic construct
GGAGNDALV

SEQ ID NO: 2688 - protein, 9 aa, synthetic construct
GGPGDDTLD

SEQ ID NO: 2689 - protein, 9 aa, synthetic construct
GGTGDDRLY

SEQ ID NO: 2690 - protein, 9 aa, synthetic construct
GGSGDDILD

SEQ ID NO: 2691 - protein, 9 aa, synthetic construct
GGGGADILR

SEQ ID NO: 2692 - protein, 9 aa, synthetic construct
GGSGDDSLA

SEQ ID NO: 2693 - protein, 9 aa, synthetic construct
GGGGNDTLH

SEQ ID NO: 2694 - protein, 9 aa, synthetic construct
GGEGADTLE

SEQ ID NO: 2695 - protein, 9 aa, synthetic construct
GGDGDDILS

SEQ ID NO: 2696 - protein, 9 aa, synthetic construct
GGLGADTMN

SEQ ID NO: 2697 - protein, 9 aa, synthetic construct
GGAGDDVYY

SEQ ID NO: 2698 - protein, 9 aa, synthetic construct
GGAGADTIV

SEQ ID NO: 2699 - protein, 9 aa, synthetic construct
GGGGNDILD

SEQ ID NO: 2700 - protein, 9 aa, synthetic construct
GGRGNDILT

SEQ ID NO: 2701 - protein, 9 aa, synthetic construct
GGAGTDTAD

SEQ ID NO: 2702 - protein, 9 aa, synthetic construct
GGAGDDLIF

SEQ ID NO: 2703 - protein, 9 aa, synthetic construct
GGGGADLFI

SEQ ID NO: 2704 - protein, 9 aa, synthetic construct
GGLGDDALR

SEQ ID NO: 2705 - protein, 9 aa, synthetic construct
GGSGNDILE

SEQ ID NO: 2706 - protein, 9 aa, synthetic construct
GGAGNDSLM

SEQ ID NO: 2707 - protein, 9 aa, synthetic construct
GGNGDDILI

SEQ ID NO: 2708 - protein, 9 aa, synthetic construct
GGAGFDILN

SEQ ID NO: 2709 - protein, 9 aa, synthetic construct
GGTGDDILS

SEQ ID NO: 2710 - protein, 9 aa, synthetic construct
GGGGSDTIR

SEQ ID NO: 2711 - protein, 9 aa, synthetic construct
GGTGADILT

SEQ ID NO: 2712 - protein, 9 aa, synthetic construct
GGEGNDTIF

SEQ ID NO: 2713 - protein, 9 aa, synthetic construct
GGRGNDLIS

SEQ ID NO: 2714 - protein, 9 aa, synthetic construct
GGSGDDTLQ

SEQ ID NO: 2715 - protein, 9 aa, synthetic construct
GGSGDDLFY

SEQ ID NO: 2716 - protein, 9 aa, synthetic construct
GGEGDDILN

SEQ ID NO: 2717 - protein, 9 aa, synthetic construct
GGLGDDVFV

SEQ ID NO: 2718 - protein, 9 aa, synthetic construct
GGSGNDVLA

SEQ ID NO: 2719 - protein, 9 aa, synthetic construct
GGQGDDTLD

SEQ ID NO: 2720 - protein, 9 aa, synthetic construct
GGRGNDLLA

SEQ ID NO: 2721 - protein, 9 aa, synthetic construct
GGDGNDQLY

SEQ ID NO: 2722 - protein, 9 aa, synthetic construct
GGGGRDRMV

SEQ ID NO: 2723 - protein, 9 aa, synthetic construct
GGIGNDTLF

SEQ ID NO: 2724 - protein, 9 aa, synthetic construct
GGGGADSLY

SEQ ID NO: 2725 - protein, 9 aa, synthetic construct
GGKGNDILK

SEQ ID NO: 2726 - protein, 9 aa, synthetic construct
GGLGNDVYV

SEQ ID NO: 2727 - protein, 9 aa, synthetic construct
GGNGNDRIY

SEQ ID NO: 2728 - protein, 9 aa, synthetic construct
GGDGDDLLY

SEQ ID NO: 2729 - protein, 9 aa, synthetic construct
GGDGADHIA

SEQ ID NO: 2730 - protein, 9 aa, synthetic construct
GGGGADKLL

SEQ ID NO: 2731 - protein, 9 aa, synthetic construct
GGLGDDSYV

SEQ ID NO: 2732 - protein, 9 aa, synthetic construct
GGAGNDIFY

SEQ ID NO: 2733 - protein, 9 aa, synthetic construct
GGTGNDWLD

SEQ ID NO: 2734 - protein, 9 aa, synthetic construct
GGTGDDTLK

SEQ ID NO: 2735 - protein, 9 aa, synthetic construct
GGNGNDQLF

SEQ ID NO: 2736 - protein, 9 aa, synthetic construct
GGRGDDTLE

SEQ ID NO: 2737 - protein, 9 aa, synthetic construct
GGDGNDILL

SEQ ID NO: 2738 - protein, 9 aa, synthetic construct
GGGGIDTLI

SEQ ID NO: 2739 - protein, 9 aa, synthetic construct
GGAGEDVLF

SEQ ID NO: 2740 - protein, 9 aa, synthetic construct
GGEGNDWLD

SEQ ID NO: 2741 - protein, 9 aa, synthetic construct
GGSGADSLS

SEQ ID NO: 2742 - protein, 9 aa, synthetic construct
GGRGDDTLD

SEQ ID NO: 2743 - protein, 9 aa, synthetic construct
GGAGDDYLW

SEQ ID NO: 2744 - protein, 9 aa, synthetic construct
GGGGNDTAD

SEQ ID NO: 2745 - protein, 9 aa, synthetic construct
GGAGRDRLD

SEQ ID NO: 2746 - protein, 9 aa, synthetic construct
GGLGDDNLY

SEQ ID NO: 2747 - protein, 9 aa, synthetic construct
GGAGNDHLS

SEQ ID NO: 2748 - protein, 9 aa, synthetic construct
GGTGDDSLT

SEQ ID NO: 2749 - protein, 9 aa, synthetic construct
GGAGDDTLM

SEQ ID NO: 2750 - protein, 9 aa, synthetic construct
GGLGNDSID

SEQ ID NO: 2751 - protein, 9 aa, synthetic construct
GGLGSDFMS

SEQ ID NO: 2752 - protein, 9 aa, synthetic construct
GGDGDDLLM

SEQ ID NO: 2753 - protein, 9 aa, synthetic construct
GGTGSDTYL

SEQ ID NO: 2754 - protein, 9 aa, synthetic construct
GGQGNDTLK

SEQ ID NO: 2755 - protein, 9 aa, synthetic construct
GGDGNDILM

SEQ ID NO: 2756 - protein, 9 aa, synthetic construct
GGAGNDSII

SEQ ID NO: 2757 - protein, 9 aa, synthetic construct
GGVGDDTLA

SEQ ID NO: 2758 - protein, 9 aa, synthetic construct
GGAGTDVFL

SEQ ID NO: 2759 - protein, 9 aa, synthetic construct
GGMGDDTLN

SEQ ID NO: 2760 - protein, 9 aa, synthetic construct
GGGGADIFI

SEQ ID NO: 2761 - protein, 9 aa, synthetic construct
GGQGDDQLT

SEQ ID NO: 2762 - protein, 9 aa, synthetic construct
GGEGNDLLR

SEQ ID NO: 2763 - protein, 9 aa, synthetic construct
GGAGADQMT

SEQ ID NO: 2764 - protein, 9 aa, synthetic construct
GGEGKDNIS

SEQ ID NO: 2765 - protein, 9 aa, synthetic construct
GGDGADSID

SEQ ID NO: 2766 - protein, 9 aa, synthetic construct
GGLGNDSLF

SEQ ID NO: 2767 - protein, 9 aa, synthetic construct
GGEGNDIVD

SEQ ID NO: 2768 - protein, 9 aa, synthetic construct
GGPGRDTLF

SEQ ID NO: 2769 - protein, 9 aa, synthetic construct
GGYGSDTYV

SEQ ID NO: 2770 - protein, 9 aa, synthetic construct
GGAGFDVLS

SEQ ID NO: 2771 - protein, 9 aa, synthetic construct
GGKGNDNLD

SEQ ID NO: 2772 - protein, 9 aa, synthetic construct
GGRGADTLF

SEQ ID NO: 2773 - protein, 9 aa, synthetic construct
GGDGDDLLT

SEQ ID NO: 2774 - protein, 9 aa, synthetic construct
GGGGDDTYD

SEQ ID NO: 2775 - protein, 9 aa, synthetic construct
GGTGNDMLS

SEQ ID NO: 2776 - protein, 9 aa, synthetic construct
GGRGDDTLT

SEQ ID NO: 2777 - protein, 9 aa, synthetic construct
GGAGDDRLW

SEQ ID NO: 2778 - protein, 9 aa, synthetic construct
GGLGDDLLS

SEQ ID NO: 2779 - protein, 9 aa, synthetic construct
GGDGNDYMS

SEQ ID NO: 2780 - protein, 9 aa, synthetic construct
GGSGNDLIE

SEQ ID NO: 2781 - protein, 9 aa, synthetic construct
GGLGDDLLV

SEQ ID NO: 2782 - protein, 9 aa, synthetic construct
GGEGDDTLA

SEQ ID NO: 2783 - protein, 9 aa, synthetic construct
GGNGDDRLY

SEQ ID NO: 2784 - protein, 9 aa, synthetic construct
GGEGDDKLT

SEQ ID NO: 2785 - protein, 9 aa, synthetic construct
GGLGNDTLH

SEQ ID NO: 2786 - protein, 9 aa, synthetic construct
GGEGSDILN

SEQ ID NO: 2787 - protein, 9 aa, synthetic construct
GGGGDDYLD

SEQ ID NO: 2788 - protein, 9 aa, synthetic construct
GGEGNDVLL

SEQ ID NO: 2789 - protein, 9 aa, synthetic construct
GGAGGDTFV

SEQ ID NO: 2790 - protein, 9 aa, synthetic construct
GGLGDDRLY

SEQ ID NO: 2791 - protein, 9 aa, synthetic construct
GGAGADRMI

SEQ ID NO: 2792 - protein, 9 aa, synthetic construct
GGAGSDRFV

SEQ ID NO: 2793 - protein, 9 aa, synthetic construct
GGAGDDWID

SEQ ID NO: 2794 - protein, 9 aa, synthetic construct
GGAGNDDLD

SEQ ID NO: 2795 - protein, 9 aa, synthetic construct
GGEGNDAVA

SEQ ID NO: 2796 - protein, 9 aa, synthetic construct
GGTGDDTIS

SEQ ID NO: 2797 - protein, 9 aa, synthetic construct
GGTGDDILT

SEQ ID NO: 2798 - protein, 9 aa, synthetic construct
GGDGDDELN

SEQ ID NO: 2799 - protein, 9 aa, synthetic construct
GGGGNDLLA

SEQ ID NO: 2800 - protein, 9 aa, synthetic construct
GGEGDDTLQ

SEQ ID NO: 2801 - protein, 9 aa, synthetic construct
GGTGADTLN

SEQ ID NO: 2802 - protein, 9 aa, synthetic construct
GGAGNDSVD

SEQ ID NO: 2803 - protein, 9 aa, synthetic construct
GGNGNDHLN

SEQ ID NO: 2804 - protein, 9 aa, synthetic construct
GGDGADTIN

SEQ ID NO: 2805 - protein, 9 aa, synthetic construct
GGAGHDRFR

SEQ ID NO: 2806 - protein, 9 aa, synthetic construct
GGAGDDFLN

SEQ ID NO: 2807 - protein, 9 aa, synthetic construct
GGSGNDALD

SEQ ID NO: 2808 - protein, 9 aa, synthetic construct
GGTGQDSLA

SEQ ID NO: 2809 - protein, 9 aa, synthetic construct
GGSGDDRLY

SEQ ID NO: 2810 - protein, 9 aa, synthetic construct
GGEGDDQLY

SEQ ID NO: 2811 - protein, 9 aa, synthetic construct
GGAGEDRLS

SEQ ID NO: 2812 - protein, 9 aa, synthetic construct
GGAGADTIH

SEQ ID NO: 2813 - protein, 9 aa, synthetic construct
GGDGNDNLV

SEQ ID NO: 2814 - protein, 9 aa, synthetic construct
GGPGDDNLQ

SEQ ID NO: 2815 - protein, 9 aa, synthetic construct
GGAGDDQLY

SEQ ID NO: 2816 - protein, 9 aa, synthetic construct
GGGGSDTLR

SEQ ID NO: 2817 - protein, 9 aa, synthetic construct
GGDGNDILS

SEQ ID NO: 2818 - protein, 9 aa, synthetic construct
GGEGNDCLY

SEQ ID NO: 2819 - protein, 9 aa, synthetic construct
GGTGDDSLS

SEQ ID NO: 2820 - protein, 9 aa, synthetic construct
GGDGNDYLN

SEQ ID NO: 2821 - protein, 9 aa, synthetic construct
GGGGRDFIT

SEQ ID NO: 2822 - protein, 9 aa, synthetic construct
GGSGSDTLL

SEQ ID NO: 2823 - protein, 9 aa, synthetic construct
GGAGDDHLD

SEQ ID NO: 2824 - protein, 9 aa, synthetic construct
GGAGNDKIS

SEQ ID NO: 2825 - protein, 9 aa, synthetic construct
GGAGEDTLT

SEQ ID NO: 2826 - protein, 9 aa, synthetic construct
GGNGSDTAS

SEQ ID NO: 2827 - protein, 9 aa, synthetic construct
GGDGNDFLS

SEQ ID NO: 2828 - protein, 9 aa, synthetic construct
GGPGDDRLF

SEQ ID NO: 2829 - protein, 9 aa, synthetic construct
GGGGNDRLF

SEQ ID NO: 2830 - protein, 9 aa, synthetic construct
GGDGNDRLN

SEQ ID NO: 2831 - protein, 9 aa, synthetic construct
GGAGRDLLS

SEQ ID NO: 2832 - protein, 9 aa, synthetic construct
GGEGNDILT

SEQ ID NO: 2833 - protein, 9 aa, synthetic construct
GGDGDDVMD

SEQ ID NO: 2834 - protein, 9 aa, synthetic construct
GGEGADRFV

SEQ ID NO: 2835 - protein, 9 aa, synthetic construct
GGYGNDTLR

SEQ ID NO: 2836 - protein, 9 aa, synthetic construct
GGGGADNMR

SEQ ID NO: 2837 - protein, 9 aa, synthetic construct
GGEGNDYLE

SEQ ID NO: 2838 - protein, 9 aa, synthetic construct
GGEGSDTLL

SEQ ID NO: 2839 - protein, 9 aa, synthetic construct
GGEGNDTII

SEQ ID NO: 2840 - protein, 9 aa, synthetic construct
GGRGNDVLD

SEQ ID NO: 2841 - protein, 9 aa, synthetic construct
GGFGADQLT

SEQ ID NO: 2842 - protein, 9 aa, synthetic construct
GGEGHDTLK

SEQ ID NO: 2843 - protein, 9 aa, synthetic construct
GGDGADQLF

SEQ ID NO: 2844 - protein, 9 aa, synthetic construct
GGNGNDSLN

SEQ ID NO: 2845 - protein, 9 aa, synthetic construct
GGEGADLLD

SEQ ID NO: 2846 - protein, 9 aa, synthetic construct
GGQGDDVLY

SEQ ID NO: 2847 - protein, 9 aa, synthetic construct
GGSGADRFI

SEQ ID NO: 2848 - protein, 9 aa, synthetic construct
GGAGDDIID

SEQ ID NO: 2849 - protein, 9 aa, synthetic construct
GGDGDDVIF

SEQ ID NO: 2850 - protein, 9 aa, synthetic construct
GGLGRDVLS

SEQ ID NO: 2851 - protein, 9 aa, synthetic construct
GGKGKDILK

SEQ ID NO: 2852 - protein, 9 aa, synthetic construct
GGSGSDTYI

SEQ ID NO: 2853 - protein, 9 aa, synthetic construct
GGGGDDRLY

SEQ ID NO: 2854 - protein, 9 aa, synthetic construct
GGAGSDVFR

SEQ ID NO: 2855 - protein, 9 aa, synthetic construct
GGSGADRLF

SEQ ID NO: 2856 - protein, 9 aa, synthetic construct
GGAGNDKLA

SEQ ID NO: 2857 - protein, 9 aa, synthetic construct
GGGGKDTFV

SEQ ID NO: 2858 - protein, 9 aa, synthetic construct
GGAGNDEIY

SEQ ID NO: 2859 - protein, 9 aa, synthetic construct
GGMGNDTLD

SEQ ID NO: 2860 - protein, 9 aa, synthetic construct
GGTGNDLLE

SEQ ID NO: 2861 - protein, 9 aa, synthetic construct
GGGGSDVLI

SEQ ID NO: 2862 - protein, 9 aa, synthetic construct
GGRGADRLN

SEQ ID NO: 2863 - protein, 9 aa, synthetic construct
GGSGDDVLE

SEQ ID NO: 2864 - protein, 9 aa, synthetic construct
GGQGNDVLD

SEQ ID NO: 2865 - protein, 9 aa, synthetic construct
GGAGSDVLT

SEQ ID NO: 2866 - protein, 9 aa, synthetic construct
GGDGDDTIN

SEQ ID NO: 2867 - protein, 9 aa, synthetic construct
GGAGEDTFV

SEQ ID NO: 2868 - protein, 9 aa, synthetic construct
GGNGNDYLN

SEQ ID NO: 2869 - protein, 9 aa, synthetic construct
GGDGSDKLY

SEQ ID NO: 2870 - protein, 9 aa, synthetic construct
GGAGFDTLA

SEQ ID NO: 2871 - protein, 9 aa, synthetic construct
GGDGNDVLA

SEQ ID NO: 2872 - protein, 9 aa, synthetic construct
GGDGDDLII

SEQ ID NO: 2873 - protein, 9 aa, synthetic construct
GGLGDDILK

SEQ ID NO: 2874 - protein, 9 aa, synthetic construct
GGLGTDTAV

SEQ ID NO: 2875 - protein, 9 aa, synthetic construct
GGTGADTLS

SEQ ID NO: 2876 - protein, 9 aa, synthetic construct
GGGGRDQLV

SEQ ID NO: 2877 - protein, 9 aa, synthetic construct
GGAGDDQLT

SEQ ID NO: 2878 - protein, 9 aa, synthetic construct
GGAGNDMLR

SEQ ID NO: 2879 - protein, 9 aa, synthetic construct
GGQGDDRLI

SEQ ID NO: 2880 - protein, 9 aa, synthetic construct
GGNGNDKLF

SEQ ID NO: 2881 - protein, 9 aa, synthetic construct
GGMGRDTLD

SEQ ID NO: 2882 - protein, 9 aa, synthetic construct
GGAGNDVII

SEQ ID NO: 2883 - protein, 9 aa, synthetic construct
GGNGDDSIN

SEQ ID NO: 2884 - protein, 9 aa, synthetic construct
GGAGADDLY

SEQ ID NO: 2885 - protein, 9 aa, synthetic construct
GGEGADVLQ

SEQ ID NO: 2886 - protein, 9 aa, synthetic construct
GGGGDDKLY

SEQ ID NO: 2887 - protein, 9 aa, synthetic construct
GGAGNDQLR

SEQ ID NO: 2888 - protein, 9 aa, synthetic construct
GGAGDDYLI

SEQ ID NO: 2889 - protein, 9 aa, synthetic construct
GGSGKDVFV

SEQ ID NO: 2890 - protein, 9 aa, synthetic construct
GGAGDDRIR

SEQ ID NO: 2891 - protein, 9 aa, synthetic construct
GGKGNDTLN

SEQ ID NO: 2892 - protein, 9 aa, synthetic construct
GGGGSDIMR

SEQ ID NO: 2893 - protein, 9 aa, synthetic construct
GGNGNDVLR

SEQ ID NO: 2894 - protein, 9 aa, synthetic construct
GGSGNDVID

SEQ ID NO: 2895 - protein, 9 aa, synthetic construct
GGAGNDQLL

SEQ ID NO: 2896 - protein, 9 aa, synthetic construct
GGTGNDALT

SEQ ID NO: 2897 - protein, 9 aa, synthetic construct
GGSGSDTAS

SEQ ID NO: 2898 - protein, 9 aa, synthetic construct
GGLGRDVLT

SEQ ID NO: 2899 - protein, 9 aa, synthetic construct
GGEGDDILD

SEQ ID NO: 2900 - protein, 9 aa, synthetic construct
GGAGRDLLL

SEQ ID NO: 2901 - protein, 9 aa, synthetic construct
GGRGNDRLE

SEQ ID NO: 2902 - protein, 9 aa, synthetic construct
GGNGDDTIY

SEQ ID NO: 2903 - protein, 9 aa, synthetic construct
GGTGADILN

SEQ ID NO: 2904 - protein, 9 aa, synthetic construct
GGGGNDVLA

SEQ ID NO: 2905 - protein, 9 aa, synthetic construct
GGTGADVLR

SEQ ID NO: 2906 - protein, 9 aa, synthetic construct
GGDGADQLE

SEQ ID NO: 2907 - protein, 9 aa, synthetic construct
GGLGADTLA

SEQ ID NO: 2908 - protein, 9 aa, synthetic construct
GGAGSDILN

SEQ ID NO: 2909 - protein, 9 aa, synthetic construct
GGAGDDRFV

SEQ ID NO: 2910 - protein, 9 aa, synthetic construct
GGDGIDTAV

SEQ ID NO: 2911 - protein, 9 aa, synthetic construct
GGDGDDQLR

SEQ ID NO: 2912 - protein, 9 aa, synthetic construct
GGNGNDLLE

SEQ ID NO: 2913 - protein, 9 aa, synthetic construct
GGGGADLLY

SEQ ID NO: 2914 - protein, 9 aa, synthetic construct
GGAGADALF

SEQ ID NO: 2915 - protein, 9 aa, synthetic construct
GGEGDDYLF

SEQ ID NO: 2916 - protein, 9 aa, synthetic construct
GGAGNDMLT

SEQ ID NO: 2917 - protein, 9 aa, synthetic construct
GGDGDDLIE

SEQ ID NO: 2918 - protein, 9 aa, synthetic construct
GGAGSDTIT

SEQ ID NO: 2919 - protein, 9 aa, synthetic construct
GGQGNDILS

SEQ ID NO: 2920 - protein, 9 aa, synthetic construct
GGDGNDKLS

SEQ ID NO: 2921 - protein, 9 aa, synthetic construct
GGAGDDKIA

SEQ ID NO: 2922 - protein, 9 aa, synthetic construct
GGAGNDWLI

SEQ ID NO: 2923 - protein, 9 aa, synthetic construct
GGKGADRLV

SEQ ID NO: 2924 - protein, 9 aa, synthetic construct
GGYGGDTYL

SEQ ID NO: 2925 - protein, 9 aa, synthetic construct
GGGGNDSLY

SEQ ID NO: 2926 - protein, 9 aa, synthetic construct
GGSGDDALS

SEQ ID NO: 2927 - protein, 9 aa, synthetic construct
GGDGGDQFI

SEQ ID NO: 2928 - protein, 9 aa, synthetic construct
GGLGADRLI

SEQ ID NO: 2929 - protein, 9 aa, synthetic construct
GGTGSDTLL

SEQ ID NO: 2930 - protein, 9 aa, synthetic construct
GGKGNDQIF

SEQ ID NO: 2931 - protein, 9 aa, synthetic construct
GGDGADLLD

SEQ ID NO: 2932 - protein, 9 aa, synthetic construct
GGTGSDTLN

SEQ ID NO: 2933 - protein, 9 aa, synthetic construct
GGDGDDTFV

SEQ ID NO: 2934 - protein, 9 aa, synthetic construct
GGGGEDTFV

SEQ ID NO: 2935 - protein, 9 aa, synthetic construct
GGGGHDYLY

SEQ ID NO: 2936 - protein, 9 aa, synthetic construct
GGNGADTYV

SEQ ID NO: 2937 - protein, 9 aa, synthetic construct
GGGGNDLLV

SEQ ID NO: 2938 - protein, 9 aa, synthetic construct
GGEGDDLLY

SEQ ID NO: 2939 - protein, 9 aa, synthetic construct
GGLGNDLLT

SEQ ID NO: 2940 - protein, 9 aa, synthetic construct
GGLGNDVLV

SEQ ID NO: 2941 - protein, 9 aa, synthetic construct
GGQGNDLLR

SEQ ID NO: 2942 - protein, 9 aa, synthetic construct
GGDGSDTAS

SEQ ID NO: 2943 - protein, 9 aa, synthetic construct
GGQGNDLLS

SEQ ID NO: 2944 - protein, 9 aa, synthetic construct
GGEGDDQIE

SEQ ID NO: 2945 - protein, 9 aa, synthetic construct
GGSGADTIN

SEQ ID NO: 2946 - protein, 9 aa, synthetic construct
GGTGNDTFI

SEQ ID NO: 2947 - protein, 9 aa, synthetic construct
GGTGNDRLV

SEQ ID NO: 2948 - protein, 9 aa, synthetic construct
GGAGHDTLT

SEQ ID NO: 2949 - protein, 9 aa, synthetic construct
GGAGNDNIG

SEQ ID NO: 2950 - protein, 9 aa, synthetic construct
GGTGNDSFI

SEQ ID NO: 2951 - protein, 9 aa, synthetic construct
GGAGNDSMY

SEQ ID NO: 2952 - protein, 9 aa, synthetic construct
GGAGADTIE

SEQ ID NO: 2953 - protein, 9 aa, synthetic construct
GGSGADTMI

SEQ ID NO: 2954 - protein, 9 aa, synthetic construct
GGDGDDVLM

SEQ ID NO: 2955 - protein, 9 aa, synthetic construct
GGGGNDTIE

SEQ ID NO: 2956 - protein, 9 aa, synthetic construct
GGAGMDSLT

SEQ ID NO: 2957 - protein, 9 aa, synthetic construct
GGGGADVFL

SEQ ID NO: 2958 - protein, 9 aa, synthetic construct
GGGGADTYV

SEQ ID NO: 2959 - protein, 9 aa, synthetic construct
GGTGDDRLS

SEQ ID NO: 2960 - protein, 9 aa, synthetic construct
GGAGNDSLW

SEQ ID NO: 2961 - protein, 9 aa, synthetic construct
GGSGNDSLA

SEQ ID NO: 2962 - protein, 9 aa, synthetic construct
GGAGADRIT

SEQ ID NO: 2963 - protein, 9 aa, synthetic construct
GGSGADTLE

SEQ ID NO: 2964 - protein, 9 aa, synthetic construct
GGDGNDVIQ

SEQ ID NO: 2965 - protein, 9 aa, synthetic construct
GGLGADELQ

SEQ ID NO: 2966 - protein, 9 aa, synthetic construct
GGLGNDYLS

SEQ ID NO: 2967 - protein, 9 aa, synthetic construct
GGTGNDILV

SEQ ID NO: 2968 - protein, 9 aa, synthetic construct
GGEGDDILV

SEQ ID NO: 2969 - protein, 9 aa, synthetic construct
GGNGADRLE

SEQ ID NO: 2970 - protein, 9 aa, synthetic construct
GGAGTDSLS

SEQ ID NO: 2971 - protein, 9 aa, synthetic construct
GGAGDDVIV

SEQ ID NO: 2972 - protein, 9 aa, synthetic construct
GGDGNDLLT

SEQ ID NO: 2973 - protein, 9 aa, synthetic construct
GGVGNDLLL

SEQ ID NO: 2974 - protein, 9 aa, synthetic construct
GGDGDDRIF

SEQ ID NO: 2975 - protein, 9 aa, synthetic construct
GGDGDDTYI

SEQ ID NO: 2976 - protein, 9 aa, synthetic construct
GGEGNDSLF

SEQ ID NO: 2977 - protein, 9 aa, synthetic construct
GGAGADFLS

SEQ ID NO: 2978 - protein, 9 aa, synthetic construct
GGNGNDVLY

SEQ ID NO: 2979 - protein, 9 aa, synthetic construct
GGAGDDIMR

SEQ ID NO: 2980 - protein, 9 aa, synthetic construct
GGSGDDIFK

SEQ ID NO: 2981 - protein, 9 aa, synthetic construct
GGLGADVMI

SEQ ID NO: 2982 - protein, 9 aa, synthetic construct
GGAGIDRLT

SEQ ID NO: 2983 - protein, 9 aa, synthetic construct
GGGGNDTIA

SEQ ID NO: 2984 - protein, 9 aa, synthetic construct
GGKGNDVLN

SEQ ID NO: 2985 - protein, 9 aa, synthetic construct
GGEGDDILK

SEQ ID NO: 2986 - protein, 9 aa, synthetic construct
GGAGNDSIE

SEQ ID NO: 2987 - protein, 9 aa, synthetic construct
GGLGKDVAL

SEQ ID NO: 2988 - protein, 9 aa, synthetic construct
GGDGDDILF

SEQ ID NO: 2989 - protein, 9 aa, synthetic construct
GGIGNDMLA

SEQ ID NO: 2990 - protein, 9 aa, synthetic construct
GGGGDDVLA

SEQ ID NO: 2991 - protein, 9 aa, synthetic construct
GGVGDDVLI

SEQ ID NO: 2992 - protein, 9 aa, synthetic construct
GGDGDDSLT

SEQ ID NO: 2993 - protein, 9 aa, synthetic construct
GGAGDDVFK

SEQ ID NO: 2994 - protein, 9 aa, synthetic construct
GGFGADTYI

SEQ ID NO: 2995 - protein, 9 aa, synthetic construct
GGSGDDSLY

SEQ ID NO: 2996 - protein, 9 aa, synthetic construct
GGGGDDTLE

SEQ ID NO: 2997 - protein, 9 aa, synthetic construct
GGAGHDTLD

SEQ ID NO: 2998 - protein, 9 aa, synthetic construct
GGNGNDVVA

SEQ ID NO: 2999 - protein, 9 aa, synthetic construct
GGTGQDTLI

SEQ ID NO: 3000 - protein, 9 aa, synthetic construct
GGTGADTLF

SEQ ID NO: 3001 - protein, 9 aa, synthetic construct
GGDGSDSYV

SEQ ID NO: 3002 - protein, 9 aa, synthetic construct
GGDGDDYLS

SEQ ID NO: 3003 - protein, 9 aa, synthetic construct
GGLGDDSLT

SEQ ID NO: 3004 - protein, 9 aa, synthetic construct
GGDGADILR

SEQ ID NO: 3005 - protein, 9 aa, synthetic construct
GGLGKDTMT

SEQ ID NO: 3006 - protein, 9 aa, synthetic construct
GGDGVDTAD

SEQ ID NO: 3007 - protein, 9 aa, synthetic construct
GGNGIDILI

SEQ ID NO: 3008 - protein, 9 aa, synthetic construct
GGAGADILA

SEQ ID NO: 3009 - protein, 9 aa, synthetic construct
GGLGDDVLV

SEQ ID NO: 3010 - protein, 9 aa, synthetic construct
GGAGTDVLI

SEQ ID NO: 3011 - protein, 9 aa, synthetic construct
GGAGVDTLL

SEQ ID NO: 3012 - protein, 9 aa, synthetic construct
GGAGADIID

SEQ ID NO: 3013 - protein, 9 aa, synthetic construct
GGFGNDTLN

SEQ ID NO: 3014 - protein, 9 aa, synthetic construct
GGAGRDTID

SEQ ID NO: 3015 - protein, 9 aa, synthetic construct
GGTGSDTYR

SEQ ID NO: 3016 - protein, 9 aa, synthetic construct
GGDGYDTVS

SEQ ID NO: 3017 - protein, 9 aa, synthetic construct
GGDGNDSIS

SEQ ID NO: 3018 - protein, 9 aa, synthetic construct
GGPGADTVV

SEQ ID NO: 3019 - protein, 9 aa, synthetic construct
GGIGADTFV

SEQ ID NO: 3020 - protein, 9 aa, synthetic construct
GGAGADMLT

SEQ ID NO: 3021 - protein, 9 aa, synthetic construct
GGLGADILD

SEQ ID NO: 3022 - protein, 9 aa, synthetic construct
GGSGNDRID

SEQ ID NO: 3023 - protein, 9 aa, synthetic construct
GGAGDDNIS

SEQ ID NO: 3024 - protein, 9 aa, synthetic construct
GGAGHDEIM

SEQ ID NO: 3025 - protein, 9 aa, synthetic construct
GGMGNDLLV

SEQ ID NO: 3026 - protein, 9 aa, synthetic construct
GGDGDDWLD

SEQ ID NO: 3027 - protein, 9 aa, synthetic construct
GGSGDDSID

SEQ ID NO: 3028 - protein, 9 aa, synthetic construct
GGGGADILT

SEQ ID NO: 3029 - protein, 9 aa, synthetic construct
GGSGNDFID

SEQ ID NO: 3030 - protein, 9 aa, synthetic construct
GGAGADNLS

SEQ ID NO: 3031 - protein, 9 aa, synthetic construct
GGEGDDVID

SEQ ID NO: 3032 - protein, 9 aa, synthetic construct
GGDGADAFI

SEQ ID NO: 3033 - protein, 9 aa, synthetic construct
GGEGNDELH

SEQ ID NO: 3034 - protein, 9 aa, synthetic construct
GGEGADYLT

SEQ ID NO: 3035 - protein, 9 aa, synthetic construct
GGLGNDTVD

SEQ ID NO: 3036 - protein, 9 aa, synthetic construct
GGGGNDVFK

SEQ ID NO: 3037 - protein, 9 aa, synthetic construct
GGTGQDTIH

SEQ ID NO: 3038 - protein, 9 aa, synthetic construct
GGEGNDSLR

SEQ ID NO: 3039 - protein, 9 aa, synthetic construct
GGTGDDTIT

SEQ ID NO: 3040 - protein, 9 aa, synthetic construct
GGTGEDILE

SEQ ID NO: 3041 - protein, 9 aa, synthetic construct
GGTGDDFLY

SEQ ID NO: 3042 - protein, 9 aa, synthetic construct
GGNGADRLD

SEQ ID NO: 3043 - protein, 9 aa, synthetic construct
GGGGQDNLS

SEQ ID NO: 3044 - protein, 9 aa, synthetic construct
GGAGADSMD

SEQ ID NO: 3045 - protein, 9 aa, synthetic construct
GGDGDDKLS

SEQ ID NO: 3046 - protein, 9 aa, synthetic construct
GGPGADRLI

SEQ ID NO: 3047 - protein, 9 aa, synthetic construct
GGAGDDEIL

SEQ ID NO: 3048 - protein, 9 aa, synthetic construct
GGAGNDLIV

SEQ ID NO: 3049 - protein, 9 aa, synthetic construct
GGLGADTFR

SEQ ID NO: 3050 - protein, 9 aa, synthetic construct
GGEGDDLLA

SEQ ID NO: 3051 - protein, 9 aa, synthetic construct
GGAGDDTIA

SEQ ID NO: 3052 - protein, 9 aa, synthetic construct
GGDGNDQLR

SEQ ID NO: 3053 - protein, 9 aa, synthetic construct
GGAGADQLD

SEQ ID NO: 3054 - protein, 9 aa, synthetic construct
GGSGNDTIE

SEQ ID NO: 3055 - protein, 9 aa, synthetic construct
GGAGNDRIS

SEQ ID NO: 3056 - protein, 9 aa, synthetic construct
GGSGNDEMF

SEQ ID NO: 3057 - protein, 9 aa, synthetic construct
GGEGSDTIN

SEQ ID NO: 3058 - protein, 9 aa, synthetic construct
GGAGNDHME

SEQ ID NO: 3059 - protein, 9 aa, synthetic construct
GGTGADTMS

SEQ ID NO: 3060 - protein, 9 aa, synthetic construct
GGSGDDSLI

SEQ ID NO: 3061 - protein, 9 aa, synthetic construct
GGDGADRFV

SEQ ID NO: 3062 - protein, 9 aa, synthetic construct
GGSGEDRLT

SEQ ID NO: 3063 - protein, 9 aa, synthetic construct
GGSGSDTFK

SEQ ID NO: 3064 - protein, 9 aa, synthetic construct
GGGGDDTIT

SEQ ID NO: 3065 - protein, 9 aa, synthetic construct
GGFGADTLI

SEQ ID NO: 3066 - protein, 9 aa, synthetic construct
GGLGNDFLT

SEQ ID NO: 3067 - protein, 9 aa, synthetic construct
GGQGDDELT

SEQ ID NO: 3068 - protein, 9 aa, synthetic construct
GGSGADIFV

SEQ ID NO: 3069 - protein, 9 aa, synthetic construct
GGAGDDTFR

SEQ ID NO: 3070 - protein, 9 aa, synthetic construct
GGRGNDEIA

SEQ ID NO: 3071 - protein, 9 aa, synthetic construct
GGLGDDIYI

SEQ ID NO: 3072 - protein, 9 aa, synthetic construct
GGDGADSIL

SEQ ID NO: 3073 - protein, 9 aa, synthetic construct
GGTGNDDLR

SEQ ID NO: 3074 - protein, 9 aa, synthetic construct
GGAGNDEII

SEQ ID NO: 3075 - protein, 9 aa, synthetic construct
GGGGTDTYD

SEQ ID NO: 3076 - protein, 9 aa, synthetic construct
GGAGTDHLV

SEQ ID NO: 3077 - protein, 9 aa, synthetic construct
GGKGDDLLE

SEQ ID NO: 3078 - protein, 9 aa, synthetic construct
GGSGDDRLN

SEQ ID NO: 3079 - protein, 9 aa, synthetic construct
GGAGDDRYV

SEQ ID NO: 3080 - protein, 9 aa, synthetic construct
GGAGNDRLK

SEQ ID NO: 3081 - protein, 9 aa, synthetic construct
GGLGNDYLV

SEQ ID NO: 3082 - protein, 9 aa, synthetic construct
GGDGDDWIS

SEQ ID NO: 3083 - protein, 9 aa, synthetic construct
GGAGDDELY

SEQ ID NO: 3084 - protein, 9 aa, synthetic construct
GGKGDDILF

SEQ ID NO: 3085 - protein, 9 aa, synthetic construct
GGLGNDFLN

SEQ ID NO: 3086 - protein, 9 aa, synthetic construct
GGSGNDFLA

SEQ ID NO: 3087 - protein, 9 aa, synthetic construct
GGNGNDYLD

SEQ ID NO: 3088 - protein, 9 aa, synthetic construct
GGLGADTLF

SEQ ID NO: 3089 - protein, 9 aa, synthetic construct
GGLGNDTLM

SEQ ID NO: 3090 - protein, 9 aa, synthetic construct
GGFGHDTLI

SEQ ID NO: 3091 - protein, 9 aa, synthetic construct
GGAGRDDVN

SEQ ID NO: 3092 - protein, 9 aa, synthetic construct
GGQGSDTFY

SEQ ID NO: 3093 - protein, 9 aa, synthetic construct
GGSGNDLLY

SEQ ID NO: 3094 - protein, 9 aa, synthetic construct
GGEGNDQLQ

SEQ ID NO: 3095 - protein, 9 aa, synthetic construct
GGNGNDVLA

SEQ ID NO: 3096 - protein, 9 aa, synthetic construct
GGEGNDTIE

SEQ ID NO: 3097 - protein, 9 aa, synthetic construct
GGSGIDTLV

SEQ ID NO: 3098 - protein, 9 aa, synthetic construct
GGDGNDVMD

SEQ ID NO: 3099 - protein, 9 aa, synthetic construct
GGTGNDFID

SEQ ID NO: 3100 - protein, 9 aa, synthetic construct
GGAGNDYLH

SEQ ID NO: 3101 - protein, 9 aa, synthetic construct
GGTGADQMN

SEQ ID NO: 3102 - protein, 9 aa, synthetic construct
GGSGADILV

SEQ ID NO: 3103 - protein, 9 aa, synthetic construct
GGVGNDLLI

SEQ ID NO: 3104 - protein, 9 aa, synthetic construct
GGAGADSIL

SEQ ID NO: 3105 - protein, 9 aa, synthetic construct
GGLGADTMA

SEQ ID NO: 3106 - protein, 9 aa, synthetic construct
GGAGADLLY

SEQ ID NO: 3107 - protein, 9 aa, synthetic construct
GGRGRDLIT

SEQ ID NO: 3108 - protein, 9 aa, synthetic construct
GGLGNDQLW

SEQ ID NO: 3109 - protein, 9 aa, synthetic construct
GGAGDDVIG

SEQ ID NO: 3110 - protein, 9 aa, synthetic construct
GGGGNDMLH

SEQ ID NO: 3111 - protein, 9 aa, synthetic construct
GGSGDDFLS

SEQ ID NO: 3112 - protein, 9 aa, synthetic construct
GGQGNDLLN

SEQ ID NO: 3113 - protein, 9 aa, synthetic construct
GGDGHDVLV

SEQ ID NO: 3114 - protein, 9 aa, synthetic construct
GGFGNDTLI

SEQ ID NO: 3115 - protein, 9 aa, synthetic construct
GGQGNDKLY

SEQ ID NO: 3116 - protein, 9 aa, synthetic construct
GGAGSDTLK

SEQ ID NO: 3117 - protein, 9 aa, synthetic construct
GGAGVDTLD

SEQ ID NO: 3118 - protein, 9 aa, synthetic construct
GGEGSDRLE

SEQ ID NO: 3119 - protein, 9 aa, synthetic construct
GGLGDDTIY

SEQ ID NO: 3120 - protein, 9 aa, synthetic construct
GGQGNDILV

SEQ ID NO: 3121 - protein, 9 aa, synthetic construct
GGTGNDTVF

SEQ ID NO: 3122 - protein, 9 aa, synthetic construct
GGEGSDLYL

SEQ ID NO: 3123 - protein, 9 aa, synthetic construct
GGDGNDTFV

SEQ ID NO: 3124 - protein, 9 aa, synthetic construct
GGIGNDELD

SEQ ID NO: 3125 - protein, 9 aa, synthetic construct
GGDGADVLI

SEQ ID NO: 3126 - protein, 9 aa, synthetic construct
GGGGNDRID

SEQ ID NO: 3127 - protein, 9 aa, synthetic construct
GGTGDDVLD

SEQ ID NO: 3128 - protein, 9 aa, synthetic construct
GGDGSDTLR

SEQ ID NO: 3129 - protein, 9 aa, synthetic construct
GGAGSDLLL

SEQ ID NO: 3130 - protein, 9 aa, synthetic construct
GGTGKDTLL

SEQ ID NO: 3131 - protein, 9 aa, synthetic construct
GGGGNDRLV

SEQ ID NO: 3132 - protein, 9 aa, synthetic construct
GGSGADRLS

SEQ ID NO: 3133 - protein, 9 aa, synthetic construct
GGSGADRLV

SEQ ID NO: 3134 - protein, 9 aa, synthetic construct
GGSGADRLY

SEQ ID NO: 3135 - protein, 9 aa, synthetic construct
GGTGNDVLH

SEQ ID NO: 3136 - protein, 9 aa, synthetic construct
GGIGNDTYI

SEQ ID NO: 3137 - protein, 9 aa, synthetic construct
GGLGADVLV

SEQ ID NO: 3138 - protein, 9 aa, synthetic construct
GGDGNDHLS

SEQ ID NO: 3139 - protein, 9 aa, synthetic construct
GGFGDDTLD

SEQ ID NO: 3140 - protein, 9 aa, synthetic construct
GGTGNDVLE

SEQ ID NO: 3141 - protein, 9 aa, synthetic construct
GGGGADTLY

SEQ ID NO: 3142 - protein, 9 aa, synthetic construct
GGDGADRLF

SEQ ID NO: 3143 - protein, 9 aa, synthetic construct
GGDGDDLLH

SEQ ID NO: 3144 - protein, 9 aa, synthetic construct
GGAGDDILQ

SEQ ID NO: 3145 - protein, 9 aa, synthetic construct
GGAGRDLLT

SEQ ID NO: 3146 - protein, 9 aa, synthetic construct
GGAGSDTYR

SEQ ID NO: 3147 - protein, 9 aa, synthetic construct
GGSGNDSLM

SEQ ID NO: 3148 - protein, 9 aa, synthetic construct
GGDGNDQLD

SEQ ID NO: 3149 - protein, 9 aa, synthetic construct
GGSGSDYLY

SEQ ID NO: 3150 - protein, 9 aa, synthetic construct
GGLGDDTLR

SEQ ID NO: 3151 - protein, 9 aa, synthetic construct
GGPGHDVLR

SEQ ID NO: 3152 - protein, 9 aa, synthetic construct
GGGGRDVMI

SEQ ID NO: 3153 - protein, 9 aa, synthetic construct
GGGGADVLN

SEQ ID NO: 3154 - protein, 9 aa, synthetic construct
GGRGNDYLY

SEQ ID NO: 3155 - protein, 9 aa, synthetic construct
GGGGSDTLT

SEQ ID NO: 3156 - protein, 9 aa, synthetic construct
GGAGADTLW

SEQ ID NO: 3157 - protein, 9 aa, synthetic construct
GGTGNDSIT

SEQ ID NO: 3158 - protein, 9 aa, synthetic construct
GGTGSDRLD

SEQ ID NO: 3159 - protein, 9 aa, synthetic construct
GGDGNDNLS

SEQ ID NO: 3160 - protein, 9 aa, synthetic construct
GGAGDDLFV

SEQ ID NO: 3161 - protein, 9 aa, synthetic construct
GGAGSDSLT

SEQ ID NO: 3162 - protein, 9 aa, synthetic construct
GGAGVDTAV

SEQ ID NO: 3163 - protein, 9 aa, synthetic construct
GGWGDDKLF

SEQ ID NO: 3164 - protein, 9 aa, synthetic construct
GGRGNDVFV

SEQ ID NO: 3165 - protein, 9 aa, synthetic construct
GGEGDDTYI

SEQ ID NO: 3166 - protein, 9 aa, synthetic construct
GGSGFDILN

SEQ ID NO: 3167 - protein, 9 aa, synthetic construct
GGDGADVLD

SEQ ID NO: 3168 - protein, 9 aa, synthetic construct
GGLGDDVLF

SEQ ID NO: 3169 - protein, 9 aa, synthetic construct
GGIGRDTLV

SEQ ID NO: 3170 - protein, 9 aa, synthetic construct
GGDGNDIYV

SEQ ID NO: 3171 - protein, 9 aa, synthetic construct
GGLGNDILQ

SEQ ID NO: 3172 - protein, 9 aa, synthetic construct
GGQGNDHLS

SEQ ID NO: 3173 - protein, 9 aa, synthetic construct
GGNGSDTLD

SEQ ID NO: 3174 - protein, 9 aa, synthetic construct
GGAGTDTVS

SEQ ID NO: 3175 - protein, 9 aa, synthetic construct
GGRGDDRLV

SEQ ID NO: 3176 - protein, 9 aa, synthetic construct
GGSGNDWIS

SEQ ID NO: 3177 - protein, 9 aa, synthetic construct
GGDGSDTLL

SEQ ID NO: 3178 - protein, 9 aa, synthetic construct
GGLGSDTFV

SEQ ID NO: 3179 - protein, 9 aa, synthetic construct
GGLGDDVYV

SEQ ID NO: 3180 - protein, 9 aa, synthetic construct
GGIGADSLI

SEQ ID NO: 3181 - protein, 9 aa, synthetic construct
GGDGEDTLN

SEQ ID NO: 3182 - protein, 9 aa, synthetic construct
GGAGADKLI

SEQ ID NO: 3183 - protein, 9 aa, synthetic construct
GGTGDDALS

SEQ ID NO: 3184 - protein, 9 aa, synthetic construct
GGAGADTMY

SEQ ID NO: 3185 - protein, 9 aa, synthetic construct
GGTGADSLS

SEQ ID NO: 3186 - protein, 9 aa, synthetic construct
GGEGDDTYD

SEQ ID NO: 3187 - protein, 9 aa, synthetic construct
GGAGNDSMT

SEQ ID NO: 3188 - protein, 9 aa, synthetic construct
GGLGADHLW

SEQ ID NO: 3189 - protein, 9 aa, synthetic construct
GGAGRDRLY

SEQ ID NO: 3190 - protein, 9 aa, synthetic construct
GGHGNDRLY

SEQ ID NO: 3191 - protein, 9 aa, synthetic construct
GGAGSDSLY

SEQ ID NO: 3192 - protein, 9 aa, synthetic construct
GGSGDDILL

SEQ ID NO: 3193 - protein, 9 aa, synthetic construct
GGTGSDVFR

SEQ ID NO: 3194 - protein, 9 aa, synthetic construct
GGVGNDTFV

SEQ ID NO: 3195 - protein, 9 aa, synthetic construct
GGIGADRLF

SEQ ID NO: 3196 - protein, 9 aa, synthetic construct
GGIGDDTLD

SEQ ID NO: 3197 - protein, 9 aa, synthetic construct
GGEGQDTLE

SEQ ID NO: 3198 - protein, 9 aa, synthetic construct
GGDGDDKLD

SEQ ID NO: 3199 - protein, 9 aa, synthetic construct
GGNGNDFIN

SEQ ID NO: 3200 - protein, 9 aa, synthetic construct
GGLGNDQLF

SEQ ID NO: 3201 - protein, 9 aa, synthetic construct
GGGGNDKLI

SEQ ID NO: 3202 - protein, 9 aa, synthetic construct
GGNGNDYLE

SEQ ID NO: 3203 - protein, 9 aa, synthetic construct
GGDGNDWLE

SEQ ID NO: 3204 - protein, 9 aa, synthetic construct
GGGGNDSIS

SEQ ID NO: 3205 - protein, 9 aa, synthetic construct
GGSGDDLID

SEQ ID NO: 3206 - protein, 9 aa, synthetic construct
GGFGNDTLT

SEQ ID NO: 3207 - protein, 9 aa, synthetic construct
GGFGADLLD

SEQ ID NO: 3208 - protein, 9 aa, synthetic construct
GGAGNDVIG

SEQ ID NO: 3209 - protein, 9 aa, synthetic construct
GGAGNDTYH

SEQ ID NO: 3210 - protein, 9 aa, synthetic construct
GGKGSDDIS

SEQ ID NO: 3211 - protein, 9 aa, synthetic construct
GGGGADTLK

SEQ ID NO: 3212 - protein, 9 aa, synthetic construct
GGKGDDIYV

SEQ ID NO: 3213 - protein, 9 aa, synthetic construct
GGLGADVFA

SEQ ID NO: 3214 - protein, 9 aa, synthetic construct
GGGGADTIS

SEQ ID NO: 3215 - protein, 9 aa, synthetic construct
GGDGADVFR

SEQ ID NO: 3216 - protein, 9 aa, synthetic construct
GGEGADNFV

SEQ ID NO: 3217 - protein, 9 aa, synthetic construct
GGSGEDSLY

SEQ ID NO: 3218 - protein, 9 aa, synthetic construct
GGQGDDSIS

SEQ ID NO: 3219 - protein, 9 aa, synthetic construct
GGLGADTVY

SEQ ID NO: 3220 - protein, 9 aa, synthetic construct
GGMGNDTIY

SEQ ID NO: 3221 - protein, 9 aa, synthetic construct
GGNGDDILF

SEQ ID NO: 3222 - protein, 9 aa, synthetic construct
GGGGRDVLD

SEQ ID NO: 3223 - protein, 9 aa, synthetic construct
GGEGDDHMS

SEQ ID NO: 3224 - protein, 9 aa, synthetic construct
GGLGADLLV

SEQ ID NO: 3225 - protein, 9 aa, synthetic construct
GGTGDDYLD

SEQ ID NO: 3226 - protein, 9 aa, synthetic construct
GGSGNDYIY

SEQ ID NO: 3227 - protein, 9 aa, synthetic construct
GGSGDDILY

SEQ ID NO: 3228 - protein, 9 aa, synthetic construct
GGAGNDFLN

SEQ ID NO: 3229 - protein, 9 aa, synthetic construct
GGAGNDDLH

SEQ ID NO: 3230 - protein, 9 aa, synthetic construct
GGAGSDVLV

SEQ ID NO: 3231 - protein, 9 aa, synthetic construct
GGAGRDTLA

SEQ ID NO: 3232 - protein, 9 aa, synthetic construct
GGLGDDRLE

SEQ ID NO: 3233 - protein, 9 aa, synthetic construct
GGSGNDVLQ

SEQ ID NO: 3234 - protein, 9 aa, synthetic construct
GGAGRDLLN

SEQ ID NO: 3235 - protein, 9 aa, synthetic construct
GGHGSDTLD

SEQ ID NO: 3236 - protein, 9 aa, synthetic construct
GGTGNDYLN

SEQ ID NO: 3237 - protein, 9 aa, synthetic construct
GGAGADIFK

SEQ ID NO: 3238 - protein, 9 aa, synthetic construct
GGAGHDVLR

SEQ ID NO: 3239 - protein, 9 aa, synthetic construct
GGRGDDVLN

SEQ ID NO: 3240 - protein, 9 aa, synthetic construct
GGDGDDVIG

SEQ ID NO: 3241 - protein, 9 aa, synthetic construct
GGTGQDTLT

SEQ ID NO: 3242 - protein, 9 aa, synthetic construct
GGDGNDILA

SEQ ID NO: 3243 - protein, 9 aa, synthetic construct
GGAGDDTIR

SEQ ID NO: 3244 - protein, 9 aa, synthetic construct
GGIGNDYID

SEQ ID NO: 3245 - protein, 9 aa, synthetic construct
GGEGSDTLR

SEQ ID NO: 3246 - protein, 9 aa, synthetic construct
GGNGNDKLI

SEQ ID NO: 3247 - protein, 9 aa, synthetic construct
GGEGSDTLT

SEQ ID NO: 3248 - protein, 9 aa, synthetic construct
GGDGNDALH

SEQ ID NO: 3249 - protein, 9 aa, synthetic construct
GGKGDDTLY

SEQ ID NO: 3250 - protein, 9 aa, synthetic construct
GGAGADSIT

SEQ ID NO: 3251 - protein, 9 aa, synthetic construct
GGDGNDRLA

SEQ ID NO: 3252 - protein, 9 aa, synthetic construct
GGGGDDRLL

SEQ ID NO: 3253 - protein, 9 aa, synthetic construct
GGAGADVLM

SEQ ID NO: 3254 - protein, 9 aa, synthetic construct
GGSGEDILI

SEQ ID NO: 3255 - protein, 9 aa, synthetic construct
GGYGNDTLL

SEQ ID NO: 3256 - protein, 9 aa, synthetic construct
GGDGNDFIS

SEQ ID NO: 3257 - protein, 9 aa, synthetic construct
GGRGNDVVS

SEQ ID NO: 3258 - protein, 9 aa, synthetic construct
GGAGADSFL

SEQ ID NO: 3259 - protein, 9 aa, synthetic construct
GGYGNDVLN

SEQ ID NO: 3260 - protein, 9 aa, synthetic construct
GGLGADTLR

SEQ ID NO: 3261 - protein, 9 aa, synthetic construct
GGEGNDSLT

SEQ ID NO: 3262 - protein, 9 aa, synthetic construct
GGSGNDVLM

SEQ ID NO: 3263 - protein, 9 aa, synthetic construct
GGRGNDLLD

SEQ ID NO: 3264 - protein, 9 aa, synthetic construct
GGNGNDVLE

SEQ ID NO: 3265 - protein, 9 aa, synthetic construct
GGNGDDILR

SEQ ID NO: 3266 - protein, 9 aa, synthetic construct
GGGGDDQIQ

SEQ ID NO: 3267 - protein, 9 aa, synthetic construct
GGRGNDLLS

SEQ ID NO: 3268 - protein, 9 aa, synthetic construct
GGTGNDIID

SEQ ID NO: 3269 - protein, 9 aa, synthetic construct
GGSGNDALY

SEQ ID NO: 3270 - protein, 9 aa, synthetic construct
GGSGNDVLL

SEQ ID NO: 3271 - protein, 9 aa, synthetic construct
GGDGADTII

SEQ ID NO: 3272 - protein, 9 aa, synthetic construct
GGDGNDALT

SEQ ID NO: 3273 - protein, 9 aa, synthetic construct
GGEGNDILY

SEQ ID NO: 3274 - protein, 9 aa, synthetic construct
GGLGADTLK

SEQ ID NO: 3275 - protein, 9 aa, synthetic construct
GGTGNDTIH

SEQ ID NO: 3276 - protein, 9 aa, synthetic construct
GGDGNDALS

SEQ ID NO: 3277 - protein, 9 aa, synthetic construct
GGAGADVLK

SEQ ID NO: 3278 - protein, 9 aa, synthetic construct
GGDGDDHLY

SEQ ID NO: 3279 - protein, 9 aa, synthetic construct
GGIGDDTYV

SEQ ID NO: 3280 - protein, 9 aa, synthetic construct
GGEGDDSLY

SEQ ID NO: 3281 - protein, 9 aa, synthetic construct
GGAGADTFT

SEQ ID NO: 3282 - protein, 9 aa, synthetic construct
GGKGVDTLR

SEQ ID NO: 3283 - protein, 9 aa, synthetic construct
GGNGDDTYI

SEQ ID NO: 3284 - protein, 9 aa, synthetic construct
GGEGNDILH

SEQ ID NO: 3285 - protein, 9 aa, synthetic construct
GGSGNDYLE

SEQ ID NO: 3286 - protein, 9 aa, synthetic construct
GGTGRDTLN

SEQ ID NO: 3287 - protein, 9 aa, synthetic construct
GGAGNDYMV

SEQ ID NO: 3288 - protein, 9 aa, synthetic construct
GGDGSDILF

SEQ ID NO: 3289 - protein, 9 aa, synthetic construct
GGTGADRMI

SEQ ID NO: 3290 - protein, 9 aa, synthetic construct
GGGGADQLF

SEQ ID NO: 3291 - protein, 9 aa, synthetic construct
GGDGDDELH

SEQ ID NO: 3292 - protein, 9 aa, synthetic construct
GGTGNDVID

SEQ ID NO: 3293 - protein, 9 aa, synthetic construct
GGAGADQLN

SEQ ID NO: 3294 - protein, 9 aa, synthetic construct
GGAGRDVLS

SEQ ID NO: 3295 - protein, 9 aa, synthetic construct
GGTGNDKLD

SEQ ID NO: 3296 - protein, 9 aa, synthetic construct
GGLGNDKLT

SEQ ID NO: 3297 - protein, 9 aa, synthetic construct
GGRGNDRLF

SEQ ID NO: 3298 - protein, 9 aa, synthetic construct
GGEGNDSLG

SEQ ID NO: 3299 - protein, 9 aa, synthetic construct
GGRGSDRMT

SEQ ID NO: 3300 - protein, 9 aa, synthetic construct
GGFGNDILR

SEQ ID NO: 3301 - protein, 9 aa, synthetic construct
GGAGVDRLL

SEQ ID NO: 3302 - protein, 9 aa, synthetic construct
GGGGDDRLE

SEQ ID NO: 3303 - protein, 9 aa, synthetic construct
GGAGDDYLF

SEQ ID NO: 3304 - protein, 9 aa, synthetic construct
GGRGDDVID

SEQ ID NO: 3305 - protein, 9 aa, synthetic construct
GGKGNDLLN

SEQ ID NO: 3306 - protein, 9 aa, synthetic construct
GGSGNDDLR

SEQ ID NO: 3307 - protein, 9 aa, synthetic construct
GGAGRDGLV

SEQ ID NO: 3308 - protein, 9 aa, synthetic construct
GGTGNDQLY

SEQ ID NO: 3309 - protein, 9 aa, synthetic construct
GGAGADRML

SEQ ID NO: 3310 - protein, 9 aa, synthetic construct
GGLGNDFLD

SEQ ID NO: 3311 - protein, 9 aa, synthetic construct
GGDGHDVLT

SEQ ID NO: 3312 - protein, 9 aa, synthetic construct
GGDGADSLN

SEQ ID NO: 3313 - protein, 9 aa, synthetic construct
GGTGDDRLI

SEQ ID NO: 3314 - protein, 9 aa, synthetic construct
GGGGNDKLF

SEQ ID NO: 3315 - protein, 9 aa, synthetic construct
GGTGNDRLN

SEQ ID NO: 3316 - protein, 9 aa, synthetic construct
GGLGNDILR

SEQ ID NO: 3317 - protein, 9 aa, synthetic construct
GGGGGDTFI

SEQ ID NO: 3318 - protein, 9 aa, synthetic construct
GGAGHDRLY

SEQ ID NO: 3319 - protein, 9 aa, synthetic construct
GGDGNDELV

SEQ ID NO: 3320 - protein, 9 aa, synthetic construct
GGNGDDTIE

SEQ ID NO: 3321 - protein, 9 aa, synthetic construct
GGRGKDILR

SEQ ID NO: 3322 - protein, 9 aa, synthetic construct
GGGGNDILL

SEQ ID NO: 3323 - protein, 9 aa, synthetic construct
GGKGSDTYV

SEQ ID NO: 3324 - protein, 9 aa, synthetic construct
GGIGDDTLV

SEQ ID NO: 3325 - protein, 9 aa, synthetic construct
GGAGDDTVN

SEQ ID NO: 3326 - protein, 9 aa, synthetic construct
GGTGSDTLI

SEQ ID NO: 3327 - protein, 9 aa, synthetic construct
GGEGTDTLH

SEQ ID NO: 3328 - protein, 9 aa, synthetic construct
GGFGDDALN

SEQ ID NO: 3329 - protein, 9 aa, synthetic construct
GGTGNDNLS

SEQ ID NO: 3330 - protein, 9 aa, synthetic construct
GGNGNDLLA

SEQ ID NO: 3331 - protein, 9 aa, synthetic construct
GGGGNDILN

SEQ ID NO: 3332 - protein, 9 aa, synthetic construct
GGLGADDLR

SEQ ID NO: 3333 - protein, 9 aa, synthetic construct
GGTGSDTLR

SEQ ID NO: 3334 - protein, 9 aa, synthetic construct
GGTGNDTVK

SEQ ID NO: 3335 - protein, 9 aa, synthetic construct
GGTGNDTVL

SEQ ID NO: 3336 - protein, 9 aa, synthetic construct
GGTGSDTLV

SEQ ID NO: 3337 - protein, 9 aa, synthetic construct
GGEGDDTIS

SEQ ID NO: 3338 - protein, 9 aa, synthetic construct
GGSGDDVLV

SEQ ID NO: 3339 - protein, 9 aa, synthetic construct
GGRGADSFV

SEQ ID NO: 3340 - protein, 9 aa, synthetic construct
GGDGDDTIV

SEQ ID NO: 3341 - protein, 9 aa, synthetic construct
GGPGNDVLT

SEQ ID NO: 3342 - protein, 9 aa, synthetic construct
GGVGDDTLS

SEQ ID NO: 3343 - protein, 9 aa, synthetic construct
GGNGNDTFV

SEQ ID NO: 3344 - protein, 9 aa, synthetic construct
GGNGNDTLA

SEQ ID NO: 3345 - protein, 9 aa, synthetic construct
GGTGDDYFV

SEQ ID NO: 3346 - protein, 9 aa, synthetic construct
GGSGHDTLI

SEQ ID NO: 3347 - protein, 9 aa, synthetic construct
GGTGDDVLI

SEQ ID NO: 3348 - protein, 9 aa, synthetic construct
GGDGDDRLS

SEQ ID NO: 3349 - protein, 9 aa, synthetic construct
GGGGSDTLD

SEQ ID NO: 3350 - protein, 9 aa, synthetic construct
GGKGNDIYI

SEQ ID NO: 3351 - protein, 9 aa, synthetic construct
GGGGADTID

SEQ ID NO: 3352 - protein, 9 aa, synthetic construct
GGAGADFMA

SEQ ID NO: 3353 - protein, 9 aa, synthetic construct
GGAGSDILS

SEQ ID NO: 3354 - protein, 9 aa, synthetic construct
GGAGDDQLS

SEQ ID NO: 3355 - protein, 9 aa, synthetic construct
GGEGNDLID

SEQ ID NO: 3356 - protein, 9 aa, synthetic construct
GGEGDDVLY

SEQ ID NO: 3357 - protein, 9 aa, synthetic construct
GGEGNDLIF

SEQ ID NO: 3358 - protein, 9 aa, synthetic construct
GGGGHDTLL

SEQ ID NO: 3359 - protein, 9 aa, synthetic construct
GGAGFDTLL

SEQ ID NO: 3360 - protein, 9 aa, synthetic construct
GGAGDDKLF

SEQ ID NO: 3361 - protein, 9 aa, synthetic construct
GGDGNDWLD

SEQ ID NO: 3362 - protein, 9 aa, synthetic construct
GGGGNDWLS

SEQ ID NO: 3363 - protein, 9 aa, synthetic construct
GGTGADRLE

SEQ ID NO: 3364 - protein, 9 aa, synthetic construct
GGEGNDTMA

SEQ ID NO: 3365 - protein, 9 aa, synthetic construct
GGTGMDTML

SEQ ID NO: 3366 - protein, 9 aa, synthetic construct
GGDGNDRIE

SEQ ID NO: 3367 - protein, 9 aa, synthetic construct
GGVGHDTMD

SEQ ID NO: 3368 - protein, 9 aa, synthetic construct
GGAGDDRIF

SEQ ID NO: 3369 - protein, 9 aa, synthetic construct
GGAGIDLLD

SEQ ID NO: 3370 - protein, 9 aa, synthetic construct
GGIGSDTLS

SEQ ID NO: 3371 - protein, 9 aa, synthetic construct
GGKGDDSLY

SEQ ID NO: 3372 - protein, 9 aa, synthetic construct
GGAGNDVMD

SEQ ID NO: 3373 - protein, 9 aa, synthetic construct
GGLGEDTLI

SEQ ID NO: 3374 - protein, 9 aa, synthetic construct
GGPGADTLD

SEQ ID NO: 3375 - protein, 9 aa, synthetic construct
GGNGDDTLA

SEQ ID NO: 3376 - protein, 9 aa, synthetic construct
GGAGSDVLE

SEQ ID NO: 3377 - protein, 9 aa, synthetic construct
GGAGNDFLY

SEQ ID NO: 3378 - protein, 9 aa, synthetic construct
GGAGSDFVN

SEQ ID NO: 3379 - protein, 9 aa, synthetic construct
GGDGNDMLI

SEQ ID NO: 3380 - protein, 9 aa, synthetic construct
GGTGNDALD

SEQ ID NO: 3381 - protein, 9 aa, synthetic construct
GGAGDDIFK

SEQ ID NO: 3382 - protein, 9 aa, synthetic construct
GGSGNDTMD

SEQ ID NO: 3383 - protein, 9 aa, synthetic construct
GGSGTDTLY

SEQ ID NO: 3384 - protein, 9 aa, synthetic construct
GGKGDDFLV

SEQ ID NO: 3385 - protein, 9 aa, synthetic construct
GGSGSDALY

SEQ ID NO: 3386 - protein, 9 aa, synthetic construct
GGEGDDYIE

SEQ ID NO: 3387 - protein, 9 aa, synthetic construct
GGTGGDSLD

SEQ ID NO: 3388 - protein, 9 aa, synthetic construct
GGSGDDILE

SEQ ID NO: 3389 - protein, 9 aa, synthetic construct
GGDGDDSIE

SEQ ID NO: 3390 - protein, 9 aa, synthetic construct
GGAGDDQIT

SEQ ID NO: 3391 - protein, 9 aa, synthetic construct
GGAGDDQIS

SEQ ID NO: 3392 - protein, 9 aa, synthetic construct
GGSGADTLH

SEQ ID NO: 3393 - protein, 9 aa, synthetic construct
GGMGDDLLR

SEQ ID NO: 3394 - protein, 9 aa, synthetic construct
GGQGNDRLD

SEQ ID NO: 3395 - protein, 9 aa, synthetic construct
GGTGIDTAS

SEQ ID NO: 3396 - protein, 9 aa, synthetic construct
GGAGSDQLD

SEQ ID NO: 3397 - protein, 9 aa, synthetic construct
GGAGADKLV

SEQ ID NO: 3398 - protein, 9 aa, synthetic construct
GGKGNDILF

SEQ ID NO: 3399 - protein, 9 aa, synthetic construct
GGAGADLLF

SEQ ID NO: 3400 - protein, 9 aa, synthetic construct
GGLGNDRLV

SEQ ID NO: 3401 - protein, 9 aa, synthetic construct
GGTGIDTLI

SEQ ID NO: 3402 - protein, 9 aa, synthetic construct
GGAGSDLMI

SEQ ID NO: 3403 - protein, 9 aa, synthetic construct
GGQGNDSLD

SEQ ID NO: 3404 - protein, 9 aa, synthetic construct
GGPGRDVFV

SEQ ID NO: 3405 - protein, 9 aa, synthetic construct
GGDGADRLY

SEQ ID NO: 3406 - protein, 9 aa, synthetic construct
GGAGNDTML

SEQ ID NO: 3407 - protein, 9 aa, synthetic construct
GGDGDDVIS

SEQ ID NO: 3408 - protein, 9 aa, synthetic construct
GGEGNDDLF

SEQ ID NO: 3409 - protein, 9 aa, synthetic construct
GGDGDDYIA

SEQ ID NO: 3410 - protein, 9 aa, synthetic construct
GGLGNDRLD

SEQ ID NO: 3411 - protein, 9 aa, synthetic construct
GGQGNDLMN

SEQ ID NO: 3412 - protein, 9 aa, synthetic construct
GGAGNDELV

SEQ ID NO: 3413 - protein, 9 aa, synthetic construct
GGGGRDTLE

SEQ ID NO: 3414 - protein, 9 aa, synthetic construct
GGQGNDSLL

SEQ ID NO: 3415 - protein, 9 aa, synthetic construct
GGLGNDVFV

SEQ ID NO: 3416 - protein, 9 aa, synthetic construct
GGAGNDTFY

SEQ ID NO: 3417 - protein, 9 aa, synthetic construct
GGEGDDHLY

SEQ ID NO: 3418 - protein, 9 aa, synthetic construct
GGAGNDVFD

SEQ ID NO: 3419 - protein, 9 aa, synthetic construct
GGAGNDVFA

SEQ ID NO: 3420 - protein, 9 aa, synthetic construct
GGEGKDTYD

SEQ ID NO: 3421 - protein, 9 aa, synthetic construct
GGGGADTLH

SEQ ID NO: 3422 - protein, 9 aa, synthetic construct
GGTGADLFR

SEQ ID NO: 3423 - protein, 9 aa, synthetic construct
GGEGNDTIS

SEQ ID NO: 3424 - protein, 9 aa, synthetic construct
GGSGQDRLT

SEQ ID NO: 3425 - protein, 9 aa, synthetic construct
GGDGNDVIS

SEQ ID NO: 3426 - protein, 9 aa, synthetic construct
GGAGSDRLL

SEQ ID NO: 3427 - protein, 9 aa, synthetic construct
GGAGDDLIV

SEQ ID NO: 3428 - protein, 9 aa, synthetic construct
GGEGADDIG

SEQ ID NO: 3429 - protein, 9 aa, synthetic construct
GGQGNDTIL

SEQ ID NO: 3430 - protein, 9 aa, synthetic construct
GGDGNDNLF

SEQ ID NO: 3431 - protein, 9 aa, synthetic construct
GGTGKDVLT

SEQ ID NO: 3432 - protein, 9 aa, synthetic construct
GGNGDDVIT

SEQ ID NO: 3433 - protein, 9 aa, synthetic construct
GGEGADVMV

SEQ ID NO: 3434 - protein, 9 aa, synthetic construct
GGAGDDLIS

SEQ ID NO: 3435 - protein, 9 aa, synthetic construct
GGLGNDQLH

SEQ ID NO: 3436 - protein, 9 aa, synthetic construct
GGAGNDTVT

SEQ ID NO: 3437 - protein, 9 aa, synthetic construct
GGAGNDRMT

SEQ ID NO: 3438 - protein, 9 aa, synthetic construct
GGDGADLLL

SEQ ID NO: 3439 - protein, 9 aa, synthetic construct
GGAGNDRIN

SEQ ID NO: 3440 - protein, 9 aa, synthetic construct
GGSGNDTFK

SEQ ID NO: 3441 - protein, 9 aa, synthetic construct
GGQGADRVY

SEQ ID NO: 3442 - protein, 9 aa, synthetic construct
GGLGNDTLG

SEQ ID NO: 3443 - protein, 9 aa, synthetic construct
GGAGNDQLE

SEQ ID NO: 3444 - protein, 9 aa, synthetic construct
GGAGNDIIR

SEQ ID NO: 3445 - protein, 9 aa, synthetic construct
GGEGNDQLY

SEQ ID NO: 3446 - protein, 9 aa, synthetic construct
GGTGADTML

SEQ ID NO: 3447 - protein, 9 aa, synthetic construct
GGIGNDTIL

SEQ ID NO: 3448 - protein, 9 aa, synthetic construct
GGAGNDRLQ

SEQ ID NO: 3449 - protein, 9 aa, synthetic construct
GGGGRDELW

SEQ ID NO: 3450 - protein, 9 aa, synthetic construct
GGTGADRFI

SEQ ID NO: 3451 - protein, 9 aa, synthetic construct
GGYGNDTIT

SEQ ID NO: 3452 - protein, 9 aa, synthetic construct
GGAGNDRLH

SEQ ID NO: 3453 - protein, 9 aa, synthetic construct
GGSGSDTLF

SEQ ID NO: 3454 - protein, 9 aa, synthetic construct
GGGGNDALD

SEQ ID NO: 3455 - protein, 9 aa, synthetic construct
GGGGADSLD

SEQ ID NO: 3456 - protein, 9 aa, synthetic construct
GGAGNDIII

SEQ ID NO: 3457 - protein, 9 aa, synthetic construct
GGIGNDSLL

SEQ ID NO: 3458 - protein, 9 aa, synthetic construct
GGSGNDVIT

SEQ ID NO: 3459 - protein, 9 aa, synthetic construct
GGGGIDTAS

SEQ ID NO: 3460 - protein, 9 aa, synthetic construct
GGYGNDILI

SEQ ID NO: 3461 - protein, 9 aa, synthetic construct
GGEGIDAAR

SEQ ID NO: 3462 - protein, 9 aa, synthetic construct
GGYGNDLLD

SEQ ID NO: 3463 - protein, 9 aa, synthetic construct
GGAGNDRFR

SEQ ID NO: 3464 - protein, 9 aa, synthetic construct
GGFGNDVYI

SEQ ID NO: 3465 - protein, 9 aa, synthetic construct
GGVGNDRLY

SEQ ID NO: 3466 - protein, 9 aa, synthetic construct
GGAGNDRIA

SEQ ID NO: 3467 - protein, 9 aa, synthetic construct
GGAGNDWIE

SEQ ID NO: 3468 - protein, 9 aa, synthetic construct
GGVGNDRLS

SEQ ID NO: 3469 - protein, 9 aa, synthetic construct
GGQGADTLV

SEQ ID NO: 3470 - protein, 9 aa, synthetic construct
GGSGNDTIH

SEQ ID NO: 3471 - protein, 9 aa, synthetic construct
GGAGDDSLF

SEQ ID NO: 3472 - protein, 9 aa, synthetic construct
GGPGNDRYE

SEQ ID NO: 3473 - protein, 9 aa, synthetic construct
GGAGNDIFR

SEQ ID NO: 3474 - protein, 9 aa, synthetic construct
GGDGDDIII

SEQ ID NO: 3475 - protein, 9 aa, synthetic construct
GGAGNDIIS

SEQ ID NO: 3476 - protein, 9 aa, synthetic construct
GGVGNDSLF

SEQ ID NO: 3477 - protein, 9 aa, synthetic construct
GGQGADSLT

SEQ ID NO: 3478 - protein, 9 aa, synthetic construct
GGQGADTLD

SEQ ID NO: 3479 - protein, 9 aa, synthetic construct
GGGGNDALS

SEQ ID NO: 3480 - protein, 9 aa, synthetic construct
GGNGNDQLD

SEQ ID NO: 3481 - protein, 9 aa, synthetic construct
GGDGDDSLN

SEQ ID NO: 3482 - protein, 9 aa, synthetic construct
GGDGRDTLN

SEQ ID NO: 3483 - protein, 9 aa, synthetic construct
GGLGDDDLN

SEQ ID NO: 3484 - protein, 9 aa, synthetic construct
GGVGDDTLN

SEQ ID NO: 3485 - protein, 9 aa, synthetic construct
GGNGDDVLY

SEQ ID NO: 3486 - protein, 9 aa, synthetic construct
GGNGRDTLD

SEQ ID NO: 3487 - protein, 9 aa, synthetic construct
GGNGADILS

SEQ ID NO: 3488 - protein, 9 aa, synthetic construct
GGEGDDVLR

SEQ ID NO: 3489 - protein, 9 aa, synthetic construct
GGSGDDRLE

SEQ ID NO: 3490 - protein, 9 aa, synthetic construct
GGLGSDVLR

SEQ ID NO: 3491 - protein, 9 aa, synthetic construct
GGTGNDSLE

SEQ ID NO: 3492 - protein, 9 aa, synthetic construct
GGDGNDSIL

SEQ ID NO: 3493 - protein, 9 aa, synthetic construct
GGNGRDTLV

SEQ ID NO: 3494 - protein, 9 aa, synthetic construct
GGSGNDFLV

SEQ ID NO: 3495 - protein, 9 aa, synthetic construct
GGGGIDTFV

SEQ ID NO: 3496 - protein, 9 aa, synthetic construct
GGFGNDVLD

SEQ ID NO: 3497 - protein, 9 aa, synthetic construct
GGVGDDTLR

SEQ ID NO: 3498 - protein, 9 aa, synthetic construct
GGQGNDGLR

SEQ ID NO: 3499 - protein, 9 aa, synthetic construct
GGQGNDLID

SEQ ID NO: 3500 - protein, 9 aa, synthetic construct
GGMGDDVLR

SEQ ID NO: 3501 - protein, 9 aa, synthetic construct
GGEGNDLLN

SEQ ID NO: 3502 - protein, 9 aa, synthetic construct
GGTGKDILI

SEQ ID NO: 3503 - protein, 9 aa, synthetic construct
GGEGADVFR

SEQ ID NO: 3504 - protein, 9 aa, synthetic construct
GGRGNDVLF

SEQ ID NO: 3505 - protein, 9 aa, synthetic construct
GGNGRDILS

SEQ ID NO: 3506 - protein, 9 aa, synthetic construct
GGAGEDVLE

SEQ ID NO: 3507 - protein, 9 aa, synthetic construct
GGRGNDVLS

SEQ ID NO: 3508 - protein, 9 aa, synthetic construct
GGSGIDTAS

SEQ ID NO: 3509 - protein, 9 aa, synthetic construct
GGAGNDTFQ

SEQ ID NO: 3510 - protein, 9 aa, synthetic construct
GGGGGDTLT

SEQ ID NO: 3511 - protein, 9 aa, synthetic construct
GGVGNDILY

SEQ ID NO: 3512 - protein, 9 aa, synthetic construct
GGLGGDTLT

SEQ ID NO: 3513 - protein, 9 aa, synthetic construct
GGAGNDLYV

SEQ ID NO: 3514 - protein, 9 aa, synthetic construct
GGAGDDVVI

SEQ ID NO: 3515 - protein, 9 aa, synthetic construct
GGDGDDILQ

SEQ ID NO: 3516 - protein, 9 aa, synthetic construct
GGSGMDYAD

SEQ ID NO: 3517 - protein, 9 aa, synthetic construct
GGAGVDTFV

SEQ ID NO: 3518 - protein, 9 aa, synthetic construct
GGSGVDTAS

SEQ ID NO: 3519 - protein, 9 aa, synthetic construct
GGIGDDKLY

SEQ ID NO: 3520 - protein, 9 aa, synthetic construct
GGAGNDGLS

SEQ ID NO: 3521 - protein, 9 aa, synthetic construct
GGDGADILN

SEQ ID NO: 3522 - protein, 9 aa, synthetic construct
GGSGDDRLL

SEQ ID NO: 3523 - protein, 9 aa, synthetic construct
GGLGSDSLD

SEQ ID NO: 3524 - protein, 9 aa, synthetic construct
GGAGGDILT

SEQ ID NO: 3525 - protein, 9 aa, synthetic construct
GGEGEDTFA

SEQ ID NO: 3526 - protein, 9 aa, synthetic construct
GGTGDDVMD

SEQ ID NO: 3527 - protein, 9 aa, synthetic construct
GGMGNDMLA

SEQ ID NO: 3528 - protein, 9 aa, synthetic construct
GGAGSDQLF

SEQ ID NO: 3529 - protein, 9 aa, synthetic construct
GGEGDDLLE

SEQ ID NO: 3530 - protein, 9 aa, synthetic construct
GGLGADFID

SEQ ID NO: 3531 - protein, 9 aa, synthetic construct
GGTGADTME

SEQ ID NO: 3532 - protein, 9 aa, synthetic construct
GGKGADQLS

SEQ ID NO: 3533 - protein, 9 aa, synthetic construct
GGAGDDALQ

SEQ ID NO: 3534 - protein, 9 aa, synthetic construct
GGIGADSLF

SEQ ID NO: 3535 - protein, 9 aa, synthetic construct
GGVGQDILE

SEQ ID NO: 3536 - protein, 9 aa, synthetic construct
GGAGNDLMT

SEQ ID NO: 3537 - protein, 9 aa, synthetic construct
GGGGADILI

SEQ ID NO: 3538 - protein, 9 aa, synthetic construct
GGVGNDMLA

SEQ ID NO: 3539 - protein, 9 aa, synthetic construct
GGAGADSIS

SEQ ID NO: 3540 - protein, 9 aa, synthetic construct
GGAGDDALY

SEQ ID NO: 3541 - protein, 9 aa, synthetic construct
GGDGDDELY

SEQ ID NO: 3542 - protein, 9 aa, synthetic construct
GGEGNDRLS

SEQ ID NO: 3543 - protein, 9 aa, synthetic construct
GGEGNDVLV

SEQ ID NO: 3544 - protein, 9 aa, synthetic construct
GGNGNDLIF

SEQ ID NO: 3545 - protein, 9 aa, synthetic construct
GGLGNDRLE

SEQ ID NO: 3546 - protein, 9 aa, synthetic construct
GGLGNDRLS

SEQ ID NO: 3547 - protein, 9 aa, synthetic construct
GGAGGDKLY

SEQ ID NO: 3548 - protein, 9 aa, synthetic construct
GGTGDDVLV

SEQ ID NO: 3549 - protein, 9 aa, synthetic construct
GGKGGDSLF

SEQ ID NO: 3550 - protein, 9 aa, synthetic construct
GGSGADTIE

SEQ ID NO: 3551 - protein, 9 aa, synthetic construct
GGGGNDRIE

SEQ ID NO: 3552 - protein, 9 aa, synthetic construct
GGGGSDTLS

SEQ ID NO: 3553 - protein, 9 aa, synthetic construct
GGDGADSLT

SEQ ID NO: 3554 - protein, 9 aa, synthetic construct
GGSGADTVV

SEQ ID NO: 3555 - protein, 9 aa, synthetic construct
GGYGDDTLI

SEQ ID NO: 3556 - protein, 9 aa, synthetic construct
GGSGSDTLE

SEQ ID NO: 3557 - protein, 9 aa, synthetic construct
GGKGDDRLE

SEQ ID NO: 3558 - protein, 9 aa, synthetic construct
GGAGNDELW

SEQ ID NO: 3559 - protein, 9 aa, synthetic construct
GGVGNDYLA

SEQ ID NO: 3560 - protein, 9 aa, synthetic construct
GGVGNDYLD

SEQ ID NO: 3561 - protein, 9 aa, synthetic construct
GGEGDDTLK

SEQ ID NO: 3562 - protein, 9 aa, synthetic construct
GGTGDDLIY

SEQ ID NO: 3563 - protein, 9 aa, synthetic construct
GGSGADTIT

SEQ ID NO: 3564 - protein, 9 aa, synthetic construct
GGLGDDTYR

SEQ ID NO: 3565 - protein, 9 aa, synthetic construct
GGDGTDTLN

SEQ ID NO: 3566 - protein, 9 aa, synthetic construct
GGDGDDTFG

SEQ ID NO: 3567 - protein, 9 aa, synthetic construct
GGDGDDTIF

SEQ ID NO: 3568 - protein, 9 aa, synthetic construct
GGEGADALY

SEQ ID NO: 3569 - protein, 9 aa, synthetic construct
GGRGDDVLS

SEQ ID NO: 3570 - protein, 9 aa, synthetic construct
GGAGADSMS

SEQ ID NO: 3571 - protein, 9 aa, synthetic construct
GGDGKDTLK

SEQ ID NO: 3572 - protein, 9 aa, synthetic construct
GGDGADRIE

SEQ ID NO: 3573 - protein, 9 aa, synthetic construct
GGAGDDYLV

SEQ ID NO: 3574 - protein, 9 aa, synthetic construct
GGQGDDVLI

SEQ ID NO: 3575 - protein, 9 aa, synthetic construct
GGNGNDTIY

SEQ ID NO: 3576 - protein, 9 aa, synthetic construct
GGGGVDTLI

SEQ ID NO: 3577 - protein, 9 aa, synthetic construct
GGNGNDWLD

SEQ ID NO: 3578 - protein, 9 aa, synthetic construct
GGAGADSMI

SEQ ID NO: 3579 - protein, 9 aa, synthetic construct
GGTGRDTLL

SEQ ID NO: 3580 - protein, 9 aa, synthetic construct
GGAGSDWMV

SEQ ID NO: 3581 - protein, 9 aa, synthetic construct
GGSGSDTYL

SEQ ID NO: 3582 - protein, 9 aa, synthetic construct
GGSGDDIIY

SEQ ID NO: 3583 - protein, 9 aa, synthetic construct
GGAGNDMLA

SEQ ID NO: 3584 - protein, 9 aa, synthetic construct
GGEGDDSIQ

SEQ ID NO: 3585 - protein, 9 aa, synthetic construct
GGLGNDTYH

SEQ ID NO: 3586 - protein, 9 aa, synthetic construct
GGAGTDRLF

SEQ ID NO: 3587 - protein, 9 aa, synthetic construct
GGAGADRMA

SEQ ID NO: 3588 - protein, 9 aa, synthetic construct
GGAGNDMIY

SEQ ID NO: 3589 - protein, 9 aa, synthetic construct
GGAGDDILW

SEQ ID NO: 3590 - protein, 9 aa, synthetic construct
GGGGDDRLS

SEQ ID NO: 3591 - protein, 9 aa, synthetic construct
GGDGDDLLN

SEQ ID NO: 3592 - protein, 9 aa, synthetic construct
GGQGEDILI

SEQ ID NO: 3593 - protein, 9 aa, synthetic construct
GGSGDDLLR

SEQ ID NO: 3594 - protein, 9 aa, synthetic construct
GGPGDDVLI

SEQ ID NO: 3595 - protein, 9 aa, synthetic construct
GGAGNDRMN

SEQ ID NO: 3596 - protein, 9 aa, synthetic construct
GGDGDDALH

SEQ ID NO: 3597 - protein, 9 aa, synthetic construct
GGKGDDWLT

SEQ ID NO: 3598 - protein, 9 aa, synthetic construct
GGEGDDALH

SEQ ID NO: 3599 - protein, 9 aa, synthetic construct
GGPGDDVLD

SEQ ID NO: 3600 - protein, 9 aa, synthetic construct
GGSGDDLLS

SEQ ID NO: 3601 - protein, 9 aa, synthetic construct
GGDGADTFI

SEQ ID NO: 3602 - protein, 9 aa, synthetic construct
GGLGADVFK

SEQ ID NO: 3603 - protein, 9 aa, synthetic construct
GGAGDDGLI

SEQ ID NO: 3604 - protein, 9 aa, synthetic construct
GGGGADLLT

SEQ ID NO: 3605 - protein, 9 aa, synthetic construct
GGTGDDYLS

SEQ ID NO: 3606 - protein, 9 aa, synthetic construct
GGAGRDLFL

SEQ ID NO: 3607 - protein, 9 aa, synthetic construct
GGIGNDRLD

SEQ ID NO: 3608 - protein, 9 aa, synthetic construct
GGQGDDTIT

SEQ ID NO: 3609 - protein, 9 aa, synthetic construct
GGTGDDQLT

SEQ ID NO: 3610 - protein, 9 aa, synthetic construct
GGDGNDRLT

SEQ ID NO: 3611 - protein, 9 aa, synthetic construct
GGEGADMLY

SEQ ID NO: 3612 - protein, 9 aa, synthetic construct
GGAGSDVLF

SEQ ID NO: 3613 - protein, 9 aa, synthetic construct
GGAGRDILI

SEQ ID NO: 3614 - protein, 9 aa, synthetic construct
GGEGADRLW

SEQ ID NO: 3615 - protein, 9 aa, synthetic construct
GGSGNDEIQ

SEQ ID NO: 3616 - protein, 9 aa, synthetic construct
GGDGADQII

SEQ ID NO: 3617 - protein, 9 aa, synthetic construct
GGDGNDNIF

SEQ ID NO: 3618 - protein, 9 aa, synthetic construct
GGAGADSLM

SEQ ID NO: 3619 - protein, 9 aa, synthetic construct
GGLGNDSLL

SEQ ID NO: 3620 - protein, 9 aa, synthetic construct
GGAGNDIFI

SEQ ID NO: 3621 - protein, 9 aa, synthetic construct
GGDGDDFLY

SEQ ID NO: 3622 - protein, 9 aa, synthetic construct
GGLGADKLY

SEQ ID NO: 3623 - protein, 9 aa, synthetic construct
GGAGKDILI

SEQ ID NO: 3624 - protein, 9 aa, synthetic construct
GGTGDDWLD

SEQ ID NO: 3625 - protein, 9 aa, synthetic construct
GGRGNDTLR

SEQ ID NO: 3626 - protein, 9 aa, synthetic construct
GGEGDDNLV

SEQ ID NO: 3627 - protein, 9 aa, synthetic construct
GGNGDDTYV

SEQ ID NO: 3628 - protein, 9 aa, synthetic construct
GGTGHDTIY

SEQ ID NO: 3629 - protein, 9 aa, synthetic construct
GGRGNDELK

SEQ ID NO: 3630 - protein, 9 aa, synthetic construct
GGTGHDTLK

SEQ ID NO: 3631 - protein, 9 aa, synthetic construct
GGAGADRIE

SEQ ID NO: 3632 - protein, 9 aa, synthetic construct
GGIGDDRLE

SEQ ID NO: 3633 - protein, 9 aa, synthetic construct
GGSGNDILA

SEQ ID NO: 3634 - protein, 9 aa, synthetic construct
GGAGKDRFV

SEQ ID NO: 3635 - protein, 9 aa, synthetic construct
GGTGDDVYI

SEQ ID NO: 3636 - protein, 9 aa, synthetic construct
GGDGTDLLT

SEQ ID NO: 3637 - protein, 9 aa, synthetic construct
GGDGNDTVY

SEQ ID NO: 3638 - protein, 9 aa, synthetic construct
GGRGNDTYV

SEQ ID NO: 3639 - protein, 9 aa, synthetic construct
GGSGQDTLS

SEQ ID NO: 3640 - protein, 9 aa, synthetic construct
GGAGNDTAV

SEQ ID NO: 3641 - protein, 9 aa, synthetic construct
GGAGKDIFV

SEQ ID NO: 3642 - protein, 9 aa, synthetic construct
GGNGDDTLF

SEQ ID NO: 3643 - protein, 9 aa, synthetic construct
GGNGDDVLD

SEQ ID NO: 3644 - protein, 9 aa, synthetic construct
GGTGADTLE

SEQ ID NO: 3645 - protein, 9 aa, synthetic construct
GGTGEDALF

SEQ ID NO: 3646 - protein, 9 aa, synthetic construct
GGLGRDFLT

SEQ ID NO: 3647 - protein, 9 aa, synthetic construct
GGGGDDFLY

SEQ ID NO: 3648 - protein, 9 aa, synthetic construct
GGMGDDVYV

SEQ ID NO: 3649 - protein, 9 aa, synthetic construct
GGAGSDYLD

SEQ ID NO: 3650 - protein, 9 aa, synthetic construct
GGDGNDRID

SEQ ID NO: 3651 - protein, 9 aa, synthetic construct
GGDGNDTFR

SEQ ID NO: 3652 - protein, 9 aa, synthetic construct
GGGGNDTIV

SEQ ID NO: 3653 - protein, 9 aa, synthetic construct
GGRGDDSLS

SEQ ID NO: 3654 - protein, 9 aa, synthetic construct
GGSGSDTAD

SEQ ID NO: 3655 - protein, 9 aa, synthetic construct
GGDGKDSLY

SEQ ID NO: 3656 - protein, 9 aa, synthetic construct
GGIGNDSLS

SEQ ID NO: 3657 - protein, 9 aa, synthetic construct
GGAGGDRFV

SEQ ID NO: 3658 - protein, 9 aa, synthetic construct
GGAGDDFLY

SEQ ID NO: 3659 - protein, 9 aa, synthetic construct
GGIGNDLLN

SEQ ID NO: 3660 - protein, 9 aa, synthetic construct
GGDGDDLIN

SEQ ID NO: 3661 - protein, 9 aa, synthetic construct
GGTGNDTVD

SEQ ID NO: 3662 - protein, 9 aa, synthetic construct
GGHGNDLMN

SEQ ID NO: 3663 - protein, 9 aa, synthetic construct
GGAGSDTFF

SEQ ID NO: 3664 - protein, 9 aa, synthetic construct
GGAGDDWLI

SEQ ID NO: 3665 - protein, 9 aa, synthetic construct
GGAGSDTAV

SEQ ID NO: 3666 - protein, 9 aa, synthetic construct
GGAGGDRID

SEQ ID NO: 3667 - protein, 9 aa, synthetic construct
GGLGDDVYY

SEQ ID NO: 3668 - protein, 9 aa, synthetic construct
GGAGVDRMT

SEQ ID NO: 3669 - protein, 9 aa, synthetic construct
GGAGDDSLQ

SEQ ID NO: 3670 - protein, 9 aa, synthetic construct
GGDGSDTYL

SEQ ID NO: 3671 - protein, 9 aa, synthetic construct
GGTGDDTLQ

SEQ ID NO: 3672 - protein, 9 aa, synthetic construct
GGGGRDTLS

SEQ ID NO: 3673 - protein, 9 aa, synthetic construct
GGPGDDILI

SEQ ID NO: 3674 - protein, 9 aa, synthetic construct
GGAGNDLMI

SEQ ID NO: 3675 - protein, 9 aa, synthetic construct
GGAGRDVMT

SEQ ID NO: 3676 - protein, 9 aa, synthetic construct
GGLGNDVLF

SEQ ID NO: 3677 - protein, 9 aa, synthetic construct
GGGGDDILR

SEQ ID NO: 3678 - protein, 9 aa, synthetic construct
GGDGNDVIL

SEQ ID NO: 3679 - protein, 9 aa, synthetic construct
GGAGHDSLD

SEQ ID NO: 3680 - protein, 9 aa, synthetic construct
GGPGNDVLV

SEQ ID NO: 3681 - protein, 9 aa, synthetic construct
GGLGSDTLV

SEQ ID NO: 3682 - protein, 9 aa, synthetic construct
GGAGADNFV

SEQ ID NO: 3683 - protein, 9 aa, synthetic construct
GGLGDDILN

SEQ ID NO: 3684 - protein, 9 aa, synthetic construct
GGAGNDLLM

SEQ ID NO: 3685 - protein, 9 aa, synthetic construct
GGTGKDTFV

SEQ ID NO: 3686 - protein, 9 aa, synthetic construct
GGNGIDTLN

SEQ ID NO: 3687 - protein, 9 aa, synthetic construct
GGGGRDTLD

SEQ ID NO: 3688 - protein, 9 aa, synthetic construct
GGNGNDILE

SEQ ID NO: 3689 - protein, 9 aa, synthetic construct
GGFGNDTYV

SEQ ID NO: 3690 - protein, 9 aa, synthetic construct
GGSGDDTYI

SEQ ID NO: 3691 - protein, 9 aa, synthetic construct
GGDGNDRLH

SEQ ID NO: 3692 - protein, 9 aa, synthetic construct
GGLGNDLLQ

SEQ ID NO: 3693 - protein, 9 aa, synthetic construct
GGDGDDTVL

SEQ ID NO: 3694 - protein, 9 aa, synthetic construct
GGYGADSID

SEQ ID NO: 3695 - protein, 9 aa, synthetic construct
GGTGNDFLS

SEQ ID NO: 3696 - protein, 9 aa, synthetic construct
GGGGNDSLF

SEQ ID NO: 3697 - protein, 9 aa, synthetic construct
GGEGRDTLL

SEQ ID NO: 3698 - protein, 9 aa, synthetic construct
GGDGNDILE

SEQ ID NO: 3699 - protein, 9 aa, synthetic construct
GGAGNDHLN

SEQ ID NO: 3700 - protein, 9 aa, synthetic construct
GGAGNDVYL

SEQ ID NO: 3701 - protein, 9 aa, synthetic construct
GGAGLDIMI

SEQ ID NO: 3702 - protein, 9 aa, synthetic construct
GGNGNDTYY

SEQ ID NO: 3703 - protein, 9 aa, synthetic construct
GGAGHDSLS

SEQ ID NO: 3704 - protein, 9 aa, synthetic construct
GGDGLDWLL

SEQ ID NO: 3705 - protein, 9 aa, synthetic construct
GGDGDDYLF

SEQ ID NO: 3706 - protein, 9 aa, synthetic construct
GGPGNDTLR

SEQ ID NO: 3707 - protein, 9 aa, synthetic construct
GGDGDDQLY

SEQ ID NO: 3708 - protein, 9 aa, synthetic construct
GGVGADTLN

SEQ ID NO: 3709 - protein, 9 aa, synthetic construct
GGAGADVMA

SEQ ID NO: 3710 - protein, 9 aa, synthetic construct
GGKGRDYID

SEQ ID NO: 3711 - protein, 9 aa, synthetic construct
GGAGADVLY

SEQ ID NO: 3712 - protein, 9 aa, synthetic construct
GGQGNDTLF

SEQ ID NO: 3713 - protein, 9 aa, synthetic construct
GGAGDDRIV

SEQ ID NO: 3714 - protein, 9 aa, synthetic construct
GGAGDDTVD

SEQ ID NO: 3715 - protein, 9 aa, synthetic construct
GGTGNDLLF

SEQ ID NO: 3716 - protein, 9 aa, synthetic construct
GGAGADDLS

SEQ ID NO: 3717 - protein, 9 aa, synthetic construct
GGDGNDSLH

SEQ ID NO: 3718 - protein, 9 aa, synthetic construct
GGDGDDHLD

SEQ ID NO: 3719 - protein, 9 aa, synthetic construct
GGFGNDTLY

SEQ ID NO: 3720 - protein, 9 aa, synthetic construct
GGAGDDTMT

SEQ ID NO: 3721 - protein, 9 aa, synthetic construct
GGTGNDALS

SEQ ID NO: 3722 - protein, 9 aa, synthetic construct
GGAGDDTMS

SEQ ID NO: 3723 - protein, 9 aa, synthetic construct
GGQGYDHLT

SEQ ID NO: 3724 - protein, 9 aa, synthetic construct
GGDGDDIIG

SEQ ID NO: 3725 - protein, 9 aa, synthetic construct
GGYGADTVI

SEQ ID NO: 3726 - protein, 9 aa, synthetic construct
GGTGDDTVM

SEQ ID NO: 3727 - protein, 9 aa, synthetic construct
GGEGEDYLE

SEQ ID NO: 3728 - protein, 9 aa, synthetic construct
GGNGDDYLY

SEQ ID NO: 3729 - protein, 9 aa, synthetic construct
GGEGNDRLN

SEQ ID NO: 3730 - protein, 9 aa, synthetic construct
GGLGDDLIY

SEQ ID NO: 3731 - protein, 9 aa, synthetic construct
GGEGSDRLY

SEQ ID NO: 3732 - protein, 9 aa, synthetic construct
GGAGDDMLL

SEQ ID NO: 3733 - protein, 9 aa, synthetic construct
GGKGNDILD

SEQ ID NO: 3734 - protein, 9 aa, synthetic construct
GGSGKDTLD

SEQ ID NO: 3735 - protein, 9 aa, synthetic construct
GGGGDDTLF

SEQ ID NO: 3736 - protein, 9 aa, synthetic construct
GGNGNDVLS

SEQ ID NO: 3737 - protein, 9 aa, synthetic construct
GGGGKDTLD

SEQ ID NO: 3738 - protein, 9 aa, synthetic construct
GGDGDDVIY

SEQ ID NO: 3739 - protein, 9 aa, synthetic construct
GGQGTDSLT

SEQ ID NO: 3740 - protein, 9 aa, synthetic construct
GGAGDDSIE

SEQ ID NO: 3741 - protein, 9 aa, synthetic construct
GGTGDDSLF

SEQ ID NO: 3742 - protein, 9 aa, synthetic construct
GGAGADDLW

SEQ ID NO: 3743 - protein, 9 aa, synthetic construct
GGLGDDLLT

SEQ ID NO: 3744 - protein, 9 aa, synthetic construct
GGAGRDTFR

SEQ ID NO: 3745 - protein, 9 aa, synthetic construct
GGDGLDTMD

SEQ ID NO: 3746 - protein, 9 aa, synthetic construct
GGAGDDQLR

SEQ ID NO: 3747 - protein, 9 aa, synthetic construct
GGAGRDTVS

SEQ ID NO: 3748 - protein, 9 aa, synthetic construct
GGSGADSLL

SEQ ID NO: 3749 - protein, 9 aa, synthetic construct
GGTGADTFL

SEQ ID NO: 3750 - protein, 9 aa, synthetic construct
GGSGDDTVL

SEQ ID NO: 3751 - protein, 9 aa, synthetic construct
GGAGDDSIT

SEQ ID NO: 3752 - protein, 9 aa, synthetic construct
GGGGADTMI

SEQ ID NO: 3753 - protein, 9 aa, synthetic construct
GGDGRDTVN

SEQ ID NO: 3754 - protein, 9 aa, synthetic construct
GGGGDDSLY

SEQ ID NO: 3755 - protein, 9 aa, synthetic construct
GGTGNDILH

SEQ ID NO: 3756 - protein, 9 aa, synthetic construct
GGVGDDILN

SEQ ID NO: 3757 - protein, 9 aa, synthetic construct
GGAGNDYLA

SEQ ID NO: 3758 - protein, 9 aa, synthetic construct
GGGGDDILD

SEQ ID NO: 3759 - protein, 9 aa, synthetic construct
GGTGDDTIL

SEQ ID NO: 3760 - protein, 9 aa, synthetic construct
GGSGDDVLL

SEQ ID NO: 3761 - protein, 9 aa, synthetic construct
GGLGDDSMT

SEQ ID NO: 3762 - protein, 9 aa, synthetic construct
GGSGDDTVS

SEQ ID NO: 3763 - protein, 9 aa, synthetic construct
GGYGADLMD

SEQ ID NO: 3764 - protein, 9 aa, synthetic construct
GGFGADTLS

SEQ ID NO: 3765 - protein, 9 aa, synthetic construct
GGSGRDTLY

SEQ ID NO: 3766 - protein, 9 aa, synthetic construct
GGDGDDLLQ

SEQ ID NO: 3767 - protein, 9 aa, synthetic construct
GGDGQDSIL

SEQ ID NO: 3768 - protein, 9 aa, synthetic construct
GGRGDDTLA

SEQ ID NO: 3769 - protein, 9 aa, synthetic construct
GGTGNDLYV

SEQ ID NO: 3770 - protein, 9 aa, synthetic construct
GGLGNDTIS

SEQ ID NO: 3771 - protein, 9 aa, synthetic construct
GGKGDDYFI

SEQ ID NO: 3772 - protein, 9 aa, synthetic construct
GGLGNDTIF

SEQ ID NO: 3773 - protein, 9 aa, synthetic construct
GGDGADLLR

SEQ ID NO: 3774 - protein, 9 aa, synthetic construct
GGGGADSLQ

SEQ ID NO: 3775 - protein, 9 aa, synthetic construct
GGAGQDSLT

SEQ ID NO: 3776 - protein, 9 aa, synthetic construct
GGSGDDLLT

SEQ ID NO: 3777 - protein, 9 aa, synthetic construct
GGQGDDTLI

SEQ ID NO: 3778 - protein, 9 aa, synthetic construct
GGSGVDYIY

SEQ ID NO: 3779 - protein, 9 aa, synthetic construct
GGAGSDVLW

SEQ ID NO: 3780 - protein, 9 aa, synthetic construct
GGEGNDKLW

SEQ ID NO: 3781 - protein, 9 aa, synthetic construct
GGDGNDIIN

SEQ ID NO: 3782 - protein, 9 aa, synthetic construct
GGSGDDFLY

SEQ ID NO: 3783 - protein, 9 aa, synthetic construct
GGSGNDTLW

SEQ ID NO: 3784 - protein, 9 aa, synthetic construct
GGSGDDLLQ

SEQ ID NO: 3785 - protein, 9 aa, synthetic construct
GGDGADLLV

SEQ ID NO: 3786 - protein, 9 aa, synthetic construct
GGNGHDIIE

SEQ ID NO: 3787 - protein, 9 aa, synthetic construct
GGSGRDTIS

SEQ ID NO: 3788 - protein, 9 aa, synthetic construct
GGAGKDTLN

SEQ ID NO: 3789 - protein, 9 aa, synthetic construct
GGWGDDTLS

SEQ ID NO: 3790 - protein, 9 aa, synthetic construct
GGSGRDTLE

SEQ ID NO: 3791 - protein, 9 aa, synthetic construct
GGDGDDQVF

SEQ ID NO: 3792 - protein, 9 aa, synthetic construct
GGEGSDLFI

SEQ ID NO: 3793 - protein, 9 aa, synthetic construct
GGLGNDTFI

SEQ ID NO: 3794 - protein, 9 aa, synthetic construct
GGTGNDLMV

SEQ ID NO: 3795 - protein, 9 aa, synthetic construct
GGMGKDQMT

SEQ ID NO: 3796 - protein, 9 aa, synthetic construct
GGSGDDILN

SEQ ID NO: 3797 - protein, 9 aa, synthetic construct
GGAGDDIIG

SEQ ID NO: 3798 - protein, 9 aa, synthetic construct
GGAGKDVLY

SEQ ID NO: 3799 - protein, 9 aa, synthetic construct
GGEGNDCLF

SEQ ID NO: 3800 - protein, 9 aa, synthetic construct
GGAGTDRLE

SEQ ID NO: 3801 - protein, 9 aa, synthetic construct
GGTGNDVLM

SEQ ID NO: 3802 - protein, 9 aa, synthetic construct
GGEGRDIVD

SEQ ID NO: 3803 - protein, 9 aa, synthetic construct
GGAGNDSIA

SEQ ID NO: 3804 - protein, 9 aa, synthetic construct
GGAGLDELT

SEQ ID NO: 3805 - protein, 9 aa, synthetic construct
GGTGADMLA

SEQ ID NO: 3806 - protein, 9 aa, synthetic construct
GGEGDDSLG

SEQ ID NO: 3807 - protein, 9 aa, synthetic construct
GGSGNDDLH

SEQ ID NO: 3808 - protein, 9 aa, synthetic construct
GGNGDDVLF

SEQ ID NO: 3809 - protein, 9 aa, synthetic construct
GGSGNDDLD

SEQ ID NO: 3810 - protein, 9 aa, synthetic construct
GGIGTDTLT

SEQ ID NO: 3811 - protein, 9 aa, synthetic construct
GGGGDDTYI

SEQ ID NO: 3812 - protein, 9 aa, synthetic construct
GGLGDDILR

SEQ ID NO: 3813 - protein, 9 aa, synthetic construct
GGFGDDTIE

SEQ ID NO: 3814 - protein, 9 aa, synthetic construct
GGLGDDQIF

SEQ ID NO: 3815 - protein, 9 aa, synthetic construct
GGAGNDFLT

SEQ ID NO: 3816 - protein, 9 aa, synthetic construct
GGPGNDKLY

SEQ ID NO: 3817 - protein, 9 aa, synthetic construct
GGTGADVLT

SEQ ID NO: 3818 - protein, 9 aa, synthetic construct
GGNGDDILY

SEQ ID NO: 3819 - protein, 9 aa, synthetic construct
GGTGRDTLI

SEQ ID NO: 3820 - protein, 9 aa, synthetic construct
GGEGSDVYH

SEQ ID NO: 3821 - protein, 9 aa, synthetic construct
GGLGNDVMT

SEQ ID NO: 3822 - protein, 9 aa, synthetic construct
GGSGRDTLI

SEQ ID NO: 3823 - protein, 9 aa, synthetic construct
GGSGSDVLK

SEQ ID NO: 3824 - protein, 9 aa, synthetic construct
GGGGSDTFD

SEQ ID NO: 3825 - protein, 9 aa, synthetic construct
GGEGSDTAS

SEQ ID NO: 3826 - protein, 9 aa, synthetic construct
GGTGRDTLT

SEQ ID NO: 3827 - protein, 9 aa, synthetic construct
GGNGNDTIN

SEQ ID NO: 3828 - protein, 9 aa, synthetic construct
GGRGNDRLL

SEQ ID NO: 3829 - protein, 9 aa, synthetic construct
GGAGADALI

SEQ ID NO: 3830 - protein, 9 aa, synthetic construct
GGNGGDTLD

SEQ ID NO: 3831 - protein, 9 aa, synthetic construct
GGTGADSIS

SEQ ID NO: 3832 - protein, 9 aa, synthetic construct
GGKGDDKLY

SEQ ID NO: 3833 - protein, 9 aa, synthetic construct
GGDGVDTVS

SEQ ID NO: 3834 - protein, 9 aa, synthetic construct
GGYGNDTLI

SEQ ID NO: 3835 - protein, 9 aa, synthetic construct
GGIGDDIYV

SEQ ID NO: 3836 - protein, 9 aa, synthetic construct
GGLGSDVFV

SEQ ID NO: 3837 - protein, 9 aa, synthetic construct
GGSGDDSLL

SEQ ID NO: 3838 - protein, 9 aa, synthetic construct
GGDGNDELD

SEQ ID NO: 3839 - protein, 9 aa, synthetic construct
GGTGADTMV

SEQ ID NO: 3840 - protein, 9 aa, synthetic construct
GGAGQDVMI

SEQ ID NO: 3841 - protein, 9 aa, synthetic construct
GGAGTDLLD

SEQ ID NO: 3842 - protein, 9 aa, synthetic construct
GGTGDDTLE

SEQ ID NO: 3843 - protein, 9 aa, synthetic construct
GGRGNDAVA

SEQ ID NO: 3844 - protein, 9 aa, synthetic construct
GGVGNDILV

SEQ ID NO: 3845 - protein, 9 aa, synthetic construct
GGKGNDLLD

SEQ ID NO: 3846 - protein, 9 aa, synthetic construct
GGDGADTFA

SEQ ID NO: 3847 - protein, 9 aa, synthetic construct
GGDGDDYLN

SEQ ID NO: 3848 - protein, 9 aa, synthetic construct
GGEGDDRLN

SEQ ID NO: 3849 - protein, 9 aa, synthetic construct
GGAGNDRIL

SEQ ID NO: 3850 - protein, 9 aa, synthetic construct
GGSGSDILS

SEQ ID NO: 3851 - protein, 9 aa, synthetic construct
GGEGADRLD

SEQ ID NO: 3852 - protein, 9 aa, synthetic construct
GGDGNDFID

SEQ ID NO: 3853 - protein, 9 aa, synthetic construct
GGLGADTID

SEQ ID NO: 3854 - protein, 9 aa, synthetic construct
GGGGDDTLR

SEQ ID NO: 3855 - protein, 9 aa, synthetic construct
GGKGDDLLV

SEQ ID NO: 3856 - protein, 9 aa, synthetic construct
GGEGRDIFQ

SEQ ID NO: 3857 - protein, 9 aa, synthetic construct
GGNGDDVVS

SEQ ID NO: 3858 - protein, 9 aa, synthetic construct
GGGGDDLLV

SEQ ID NO: 3859 - protein, 9 aa, synthetic construct
GGAGADNLA

SEQ ID NO: 3860 - protein, 9 aa, synthetic construct
GGAGNDWLL

SEQ ID NO: 3861 - protein, 9 aa, synthetic construct
GGYGYDTLN

SEQ ID NO: 3862 - protein, 9 aa, synthetic construct
GGGGADRLQ

SEQ ID NO: 3863 - protein, 9 aa, synthetic construct
GGAGDDSLM

SEQ ID NO: 3864 - protein, 9 aa, synthetic construct
GGEGRDTLY

SEQ ID NO: 3865 - protein, 9 aa, synthetic construct
GGAGTDILN

SEQ ID NO: 3866 - protein, 9 aa, synthetic construct
GGAGADGLD

SEQ ID NO: 3867 - protein, 9 aa, synthetic construct
GGNGDDALF

SEQ ID NO: 3868 - protein, 9 aa, synthetic construct
GGGGADILY

SEQ ID NO: 3869 - protein, 9 aa, synthetic construct
GGLGNDLLE

SEQ ID NO: 3870 - protein, 9 aa, synthetic construct
GGGGADILD

SEQ ID NO: 3871 - protein, 9 aa, synthetic construct
GGAGDDELS

SEQ ID NO: 3872 - protein, 9 aa, synthetic construct
GGDGNDKIV

SEQ ID NO: 3873 - protein, 9 aa, synthetic construct
GGGGVDTLS

SEQ ID NO: 3874 - protein, 9 aa, synthetic construct
GGDGDDRID

SEQ ID NO: 3875 - protein, 9 aa, synthetic construct
GGDGNDTLG

SEQ ID NO: 3876 - protein, 9 aa, synthetic construct
GGLGDDLLR

SEQ ID NO: 3877 - protein, 9 aa, synthetic construct
GGVGSDWMV

SEQ ID NO: 3878 - protein, 9 aa, synthetic construct
GGEGDDALD

SEQ ID NO: 3879 - protein, 9 aa, synthetic construct
GGDGSDFYV

SEQ ID NO: 3880 - protein, 9 aa, synthetic construct
GGDGDDRIG

SEQ ID NO: 3881 - protein, 9 aa, synthetic construct
GGEGNDSIF

SEQ ID NO: 3882 - protein, 9 aa, synthetic construct
GGGGDDRLA

SEQ ID NO: 3883 - protein, 9 aa, synthetic construct
GGEGDDVLA

SEQ ID NO: 3884 - protein, 9 aa, synthetic construct
GGTGADQFV

SEQ ID NO: 3885 - protein, 9 aa, synthetic construct
GGTGDDMLD

SEQ ID NO: 3886 - protein, 9 aa, synthetic construct
GGSGNDVIR

SEQ ID NO: 3887 - protein, 9 aa, synthetic construct
GGGGSDKLW

SEQ ID NO: 3888 - protein, 9 aa, synthetic construct
GGSGIDTVF

SEQ ID NO: 3889 - protein, 9 aa, synthetic construct
GGAGADELD

SEQ ID NO: 3890 - protein, 9 aa, synthetic construct
GGDGSDLYY

SEQ ID NO: 3891 - protein, 9 aa, synthetic construct
GGAGRDILT

SEQ ID NO: 3892 - protein, 9 aa, synthetic construct
GGDGADLLI

SEQ ID NO: 3893 - protein, 9 aa, synthetic construct
GGAGNDRLW

SEQ ID NO: 3894 - protein, 9 aa, synthetic construct
GGAGQDTLF

SEQ ID NO: 3895 - protein, 9 aa, synthetic construct
GGSGNDMLF

SEQ ID NO: 3896 - protein, 9 aa, synthetic construct
GGNGDDVLR

SEQ ID NO: 3897 - protein, 9 aa, synthetic construct
GGSGNDMLT

SEQ ID NO: 3898 - protein, 9 aa, synthetic construct
GGAGRDIMS

SEQ ID NO: 3899 - protein, 9 aa, synthetic construct
GGAGNDRME

SEQ ID NO: 3900 - protein, 9 aa, synthetic construct
GGGGNDTFA

SEQ ID NO: 3901 - protein, 9 aa, synthetic construct
GGGGADSLI

SEQ ID NO: 3902 - protein, 9 aa, synthetic construct
GGVGNDSLS

SEQ ID NO: 3903 - protein, 9 aa, synthetic construct
GGSGADHFV

SEQ ID NO: 3904 - protein, 9 aa, synthetic construct
GGTGADVFV

SEQ ID NO: 3905 - protein, 9 aa, synthetic construct
GGGGSDVLY

SEQ ID NO: 3906 - protein, 9 aa, synthetic construct
GGGGADLLK

SEQ ID NO: 3907 - protein, 9 aa, synthetic construct
GGDGDDALF

SEQ ID NO: 3908 - protein, 9 aa, synthetic construct
GGAGGDVLD

SEQ ID NO: 3909 - protein, 9 aa, synthetic construct
GGDGHDTLL

SEQ ID NO: 3910 - protein, 9 aa, synthetic construct
GGAGIDRVD

SEQ ID NO: 3911 - protein, 9 aa, synthetic construct
GGGGNDVVA

SEQ ID NO: 3912 - protein, 9 aa, synthetic construct
GGAGRDILA

SEQ ID NO: 3913 - protein, 9 aa, synthetic construct
GGSGHDSLT

SEQ ID NO: 3914 - protein, 9 aa, synthetic construct
GGIGNDSLF

SEQ ID NO: 3915 - protein, 9 aa, synthetic construct
GGLGNDLLV

SEQ ID NO: 3916 - protein, 9 aa, synthetic construct
GGDGDDLLA

SEQ ID NO: 3917 - protein, 9 aa, synthetic construct
GGAGNDFVS

SEQ ID NO: 3918 - protein, 9 aa, synthetic construct
GGTGNDELK

SEQ ID NO: 3919 - protein, 9 aa, synthetic construct
GGAGADDIV

SEQ ID NO: 3920 - protein, 9 aa, synthetic construct
GGAGDDFYV

SEQ ID NO: 3921 - protein, 9 aa, synthetic construct
GGAGNDLIH

SEQ ID NO: 3922 - protein, 9 aa, synthetic construct
GGEGNDYLS

SEQ ID NO: 3923 - protein, 9 aa, synthetic construct
GGDGADTLQ

SEQ ID NO: 3924 - protein, 9 aa, synthetic construct
GGEGNDWLL

SEQ ID NO: 3925 - protein, 9 aa, synthetic construct
GGYGNDTLW

SEQ ID NO: 3926 - protein, 9 aa, synthetic construct
GGGGDDTLY

SEQ ID NO: 3927 - protein, 9 aa, synthetic construct
GGEGVDTAD

SEQ ID NO: 3928 - protein, 9 aa, synthetic construct
GGAGADDLR

SEQ ID NO: 3929 - protein, 9 aa, synthetic construct
GGSGNDELD

SEQ ID NO: 3930 - protein, 9 aa, synthetic construct
GGTGNDKLF

SEQ ID NO: 3931 - protein, 9 aa, synthetic construct
GGDGVDTLS

SEQ ID NO: 3932 - protein, 9 aa, synthetic construct
GGAGVDLLT

SEQ ID NO: 3933 - protein, 9 aa, synthetic construct
GGQGADILT

SEQ ID NO: 3934 - protein, 9 aa, synthetic construct
GGAGFDSAD

SEQ ID NO: 3935 - protein, 9 aa, synthetic construct
GGSGADFLD

SEQ ID NO: 3936 - protein, 9 aa, synthetic construct
GGTGDDRLD

SEQ ID NO: 3937 - protein, 9 aa, synthetic construct
GGAGADTFH

SEQ ID NO: 3938 - protein, 9 aa, synthetic construct
GGGGNDRIY

SEQ ID NO: 3939 - protein, 9 aa, synthetic construct
GGAGADRFL

SEQ ID NO: 3940 - protein, 9 aa, synthetic construct
GGAGADRFE

SEQ ID NO: 3941 - protein, 9 aa, synthetic construct
GGLGNDSIL

SEQ ID NO: 3942 - protein, 9 aa, synthetic construct
GGAGDDVMV

SEQ ID NO: 3943 - protein, 9 aa, synthetic construct
GGGGNDRLY

SEQ ID NO: 3944 - protein, 9 aa, synthetic construct
GGTGDDLLL

SEQ ID NO: 3945 - protein, 9 aa, synthetic construct
GGAGDDVMQ

SEQ ID NO: 3946 - protein, 9 aa, synthetic construct
GGSGADQLV

SEQ ID NO: 3947 - protein, 9 aa, synthetic construct
GGGGRDVLI

SEQ ID NO: 3948 - protein, 9 aa, synthetic construct
GGQGNDTIY

SEQ ID NO: 3949 - protein, 9 aa, synthetic construct
GGAGADVFQ

SEQ ID NO: 3950 - protein, 9 aa, synthetic construct
GGAGTDWLD

SEQ ID NO: 3951 - protein, 9 aa, synthetic construct
GGGGSDTLY

SEQ ID NO: 3952 - protein, 9 aa, synthetic construct
GGEGNDHLY

SEQ ID NO: 3953 - protein, 9 aa, synthetic construct
GGAGNDLMD

SEQ ID NO: 3954 - protein, 9 aa, synthetic construct
GGKGNDTID

SEQ ID NO: 3955 - protein, 9 aa, synthetic construct
GGMGADTLT

SEQ ID NO: 3956 - protein, 9 aa, synthetic construct
GGAGNDKLH

SEQ ID NO: 3957 - protein, 9 aa, synthetic construct
GGSGSDELY

SEQ ID NO: 3958 - protein, 9 aa, synthetic construct
GGKGNDTLS

SEQ ID NO: 3959 - protein, 9 aa, synthetic construct
GGNGDDYID

SEQ ID NO: 3960 - protein, 9 aa, synthetic construct
GGDGADILQ

SEQ ID NO: 3961 - protein, 9 aa, synthetic construct
GGGGNDTVY

SEQ ID NO: 3962 - protein, 9 aa, synthetic construct
GGAGNDTIK

SEQ ID NO: 3963 - protein, 9 aa, synthetic construct
GGGGADVID

SEQ ID NO: 3964 - protein, 9 aa, synthetic construct
GGVGADTLS

SEQ ID NO: 3965 - protein, 9 aa, synthetic construct
GGSGNDQLA

SEQ ID NO: 3966 - protein, 9 aa, synthetic construct
GGNGNDRLT

SEQ ID NO: 3967 - protein, 9 aa, synthetic construct
GGDGNDIFV

SEQ ID NO: 3968 - protein, 9 aa, synthetic construct
GGDGADRLL

SEQ ID NO: 3969 - protein, 9 aa, synthetic construct
GGGGNDLLH

SEQ ID NO: 3970 - protein, 9 aa, synthetic construct
GGAGDDTVF

SEQ ID NO: 3971 - protein, 9 aa, synthetic construct
GGAGDDVYL

SEQ ID NO: 3972 - protein, 9 aa, synthetic construct
GGVGDDVLS

SEQ ID NO: 3973 - protein, 9 aa, synthetic construct
GGDGNDLIR

SEQ ID NO: 3974 - protein, 9 aa, synthetic construct
GGTGDDSLY

SEQ ID NO: 3975 - protein, 9 aa, synthetic construct
GGSGDDTIS

SEQ ID NO: 3976 - protein, 9 aa, synthetic construct
GGDGNDSIY

SEQ ID NO: 3977 - protein, 9 aa, synthetic construct
GGNGNDTYV

SEQ ID NO: 3978 - protein, 9 aa, synthetic construct
GGYGTDFIN

SEQ ID NO: 3979 - protein, 9 aa, synthetic construct
GGSGRDLLD

SEQ ID NO: 3980 - protein, 9 aa, synthetic construct
GGGGDDVID

SEQ ID NO: 3981 - protein, 9 aa, synthetic construct
GGAGNDIYF

SEQ ID NO: 3982 - protein, 9 aa, synthetic construct
GGTGDDLLV

SEQ ID NO: 3983 - protein, 9 aa, synthetic construct
GGTGNDNLY

SEQ ID NO: 3984 - protein, 9 aa, synthetic construct
GGAGADKFD

SEQ ID NO: 3985 - protein, 9 aa, synthetic construct
GGVGRDTLI

SEQ ID NO: 3986 - protein, 9 aa, synthetic construct
GGTGDDLLS

SEQ ID NO: 3987 - protein, 9 aa, synthetic construct
GGAGADRFF

SEQ ID NO: 3988 - protein, 9 aa, synthetic construct
GGNGNDVLW

SEQ ID NO: 3989 - protein, 9 aa, synthetic construct
GGGGADELL

SEQ ID NO: 3990 - protein, 9 aa, synthetic construct
GGTGDDSLR

SEQ ID NO: 3991 - protein, 9 aa, synthetic construct
GGDGGDYLT

SEQ ID NO: 3992 - protein, 9 aa, synthetic construct
GGSGGDTLI

SEQ ID NO: 3993 - protein, 9 aa, synthetic construct
GGDGLDTID

SEQ ID NO: 3994 - protein, 9 aa, synthetic construct
GGAGGDILD

SEQ ID NO: 3995 - protein, 9 aa, synthetic construct
GGTGSDTYV

SEQ ID NO: 3996 - protein, 9 aa, synthetic construct
GGTGDDVIY

SEQ ID NO: 3997 - protein, 9 aa, synthetic construct
GGAGDDVIA

SEQ ID NO: 3998 - protein, 9 aa, synthetic construct
GGYGSDTYL

SEQ ID NO: 3999 - protein, 9 aa, synthetic construct
GGKGDDIYL

SEQ ID NO: 4000 - protein, 9 aa, synthetic construct
GGGGHDILN

SEQ ID NO: 4001 - protein, 9 aa, synthetic construct
GGQGNDLMY

SEQ ID NO: 4002 - protein, 9 aa, synthetic construct
GGAGADFLA

SEQ ID NO: 4003 - protein, 9 aa, synthetic construct
GGAGIDTLY

SEQ ID NO: 4004 - protein, 9 aa, synthetic construct
GGAGNDTMR

SEQ ID NO: 4005 - protein, 9 aa, synthetic construct
GGDGADRLS

SEQ ID NO: 4006 - protein, 9 aa, synthetic construct
GGAGDDVIF

SEQ ID NO: 4007 - protein, 9 aa, synthetic construct
GGNGADTLL

SEQ ID NO: 4008 - protein, 9 aa, synthetic construct
GGTGDDVLL

SEQ ID NO: 4009 - protein, 9 aa, synthetic construct
GGQGNDLLA

SEQ ID NO: 4010 - protein, 9 aa, synthetic construct
GGIGNDVLS

SEQ ID NO: 4011 - protein, 9 aa, synthetic construct
GGAGQDIFV

SEQ ID NO: 4012 - protein, 9 aa, synthetic construct
GGAGNDELT

SEQ ID NO: 4013 - protein, 9 aa, synthetic construct
GGDGNDSVS

SEQ ID NO: 4014 - protein, 9 aa, synthetic construct
GGDGDDLMG

SEQ ID NO: 4015 - protein, 9 aa, synthetic construct
GGGGADQLI

SEQ ID NO: 4016 - protein, 9 aa, synthetic construct
GGGGNDSID

SEQ ID NO: 4017 - protein, 9 aa, synthetic construct
GGGGADALT

SEQ ID NO: 4018 - protein, 9 aa, synthetic construct
GGAGTDTLV

SEQ ID NO: 4019 - protein, 9 aa, synthetic construct
GGGGNDIID

SEQ ID NO: 4020 - protein, 9 aa, synthetic construct
GGDGDDVIN

SEQ ID NO: 4021 - protein, 9 aa, synthetic construct
GGDGADILD

SEQ ID NO: 4022 - protein, 9 aa, synthetic construct
GGSGADRLT

SEQ ID NO: 4023 - protein, 9 aa, synthetic construct
GGTGDDSLL

SEQ ID NO: 4024 - protein, 9 aa, synthetic construct
GGAGTDTLR

SEQ ID NO: 4025 - protein, 9 aa, synthetic construct
GGIGNDTYF

SEQ ID NO: 4026 - protein, 9 aa, synthetic construct
GGAGNDLYI

SEQ ID NO: 4027 - protein, 9 aa, synthetic construct
GGEGNDRLV

SEQ ID NO: 4028 - protein, 9 aa, synthetic construct
GGAGADLLH

SEQ ID NO: 4029 - protein, 9 aa, synthetic construct
GGTGDDVIN

SEQ ID NO: 4030 - protein, 9 aa, synthetic construct
GGDGRDTLD

SEQ ID NO: 4031 - protein, 9 aa, synthetic construct
GGAGDDAVA

SEQ ID NO: 4032 - protein, 9 aa, synthetic construct
GGEGNDRLI

SEQ ID NO: 4033 - protein, 9 aa, synthetic construct
GGGGNDTLW

SEQ ID NO: 4034 - protein, 9 aa, synthetic construct
GGDGDDDLD

SEQ ID NO: 4035 - protein, 9 aa, synthetic construct
GGAGHDRLF

SEQ ID NO: 4036 - protein, 9 aa, synthetic construct
GGLGDDTVL

SEQ ID NO: 4037 - protein, 9 aa, synthetic construct
GGAGNDTMY

SEQ ID NO: 4038 - protein, 9 aa, synthetic construct
GGGGNDLIG

SEQ ID NO: 4039 - protein, 9 aa, synthetic construct
GGFGFDRIN

SEQ ID NO: 4040 - protein, 9 aa, synthetic construct
GGTGDDSIL

SEQ ID NO: 4041 - protein, 9 aa, synthetic construct
GGTGDDIYI

SEQ ID NO: 4042 - protein, 9 aa, synthetic construct
GGNGNDLLF

SEQ ID NO: 4043 - protein, 9 aa, synthetic construct
GGAGNDSMF

SEQ ID NO: 4044 - protein, 9 aa, synthetic construct
GGVGGDQLF

SEQ ID NO: 4045 - protein, 9 aa, synthetic construct
GGAGSDTLM

SEQ ID NO: 4046 - protein, 9 aa, synthetic construct
GGTGNDTIF

SEQ ID NO: 4047 - protein, 9 aa, synthetic construct
GGSGEDYVS

SEQ ID NO: 4048 - protein, 9 aa, synthetic construct
GGAGRDTLV

SEQ ID NO: 4049 - protein, 9 aa, synthetic construct
GGSGNDTVD

SEQ ID NO: 4050 - protein, 9 aa, synthetic construct
GGGGDDSLA

SEQ ID NO: 4051 - protein, 9 aa, synthetic construct
GGAGSDTIY

SEQ ID NO: 4052 - protein, 9 aa, synthetic construct
GGSGDDDIF

SEQ ID NO: 4053 - protein, 9 aa, synthetic construct
GGRGNDTIY

SEQ ID NO: 4054 - protein, 9 aa, synthetic construct
GGSGDDFIF

SEQ ID NO: 4055 - protein, 9 aa, synthetic construct
GGAGSDSMS

SEQ ID NO: 4056 - protein, 9 aa, synthetic construct
GGEGKDTLQ

SEQ ID NO: 4057 - protein, 9 aa, synthetic construct
GGIGNDLLE

SEQ ID NO: 4058 - protein, 9 aa, synthetic construct
GGIGNDLLD

SEQ ID NO: 4059 - protein, 9 aa, synthetic construct
GGGGRDLLN

SEQ ID NO: 4060 - protein, 9 aa, synthetic construct
GGGGADVLV

SEQ ID NO: 4061 - protein, 9 aa, synthetic construct
GGGGNDVLE

SEQ ID NO: 4062 - protein, 9 aa, synthetic construct
GGNGNDQLT

SEQ ID NO: 4063 - protein, 9 aa, synthetic construct
GGGGNDILM

SEQ ID NO: 4064 - protein, 9 aa, synthetic construct
GGDGFDFIN

SEQ ID NO: 4065 - protein, 9 aa, synthetic construct
GGSGNDYMH

SEQ ID NO: 4066 - protein, 9 aa, synthetic construct
GGSGNDSIS

SEQ ID NO: 4067 - protein, 9 aa, synthetic construct
GGAGNDVIA

SEQ ID NO: 4068 - protein, 9 aa, synthetic construct
GGAGNDFIR

SEQ ID NO: 4069 - protein, 9 aa, synthetic construct
GGSGNDLIG

SEQ ID NO: 4070 - protein, 9 aa, synthetic construct
GGAGADTFY

SEQ ID NO: 4071 - protein, 9 aa, synthetic construct
GGSGNDSIT

SEQ ID NO: 4072 - protein, 9 aa, synthetic construct
GGEGNDNLY

SEQ ID NO: 4073 - protein, 9 aa, synthetic construct
GGAGNDVIH

SEQ ID NO: 4074 - protein, 9 aa, synthetic construct
GGNGNDNLA

SEQ ID NO: 4075 - protein, 9 aa, synthetic construct
GGLGNDSLI

SEQ ID NO: 4076 - protein, 9 aa, synthetic construct
GGSGDDFLD

SEQ ID NO: 4077 - protein, 9 aa, synthetic construct
GGIGADTLL

SEQ ID NO: 4078 - protein, 9 aa, synthetic construct
GGNGADSLT

SEQ ID NO: 4079 - protein, 9 aa, synthetic construct
GGAGEDTVF

SEQ ID NO: 4080 - protein, 9 aa, synthetic construct
GGTGADRLT

SEQ ID NO: 4081 - protein, 9 aa, synthetic construct
GGRGSDELK

SEQ ID NO: 4082 - protein, 9 aa, synthetic construct
GGIGADTLN

SEQ ID NO: 4083 - protein, 9 aa, synthetic construct
GGTGHDTLI

SEQ ID NO: 4084 - protein, 9 aa, synthetic construct
GGDGNDFVN

SEQ ID NO: 4085 - protein, 9 aa, synthetic construct
GGSGADKLT

SEQ ID NO: 4086 - protein, 9 aa, synthetic construct
GGSGQDTLI

SEQ ID NO: 4087 - protein, 9 aa, synthetic construct
GGAGNDAVS

SEQ ID NO: 4088 - protein, 9 aa, synthetic construct
GGSGDDSIR

SEQ ID NO: 4089 - protein, 9 aa, synthetic construct
GGLGADFMA

SEQ ID NO: 4090 - protein, 9 aa, synthetic construct
GGSGADTMY

SEQ ID NO: 4091 - protein, 9 aa, synthetic construct
GGAGNDAVL

SEQ ID NO: 4092 - protein, 9 aa, synthetic construct
GGAGKDRLR

SEQ ID NO: 4093 - protein, 9 aa, synthetic construct
GGSGQDVLF

SEQ ID NO: 4094 - protein, 9 aa, synthetic construct
GGTGDDRLL

SEQ ID NO: 4095 - protein, 9 aa, synthetic construct
GGTGEDTLI

SEQ ID NO: 4096 - protein, 9 aa, synthetic construct
GGSGADSMT

SEQ ID NO: 4097 - protein, 9 aa, synthetic construct
GGSGDDFLT

SEQ ID NO: 4098 - protein, 9 aa, synthetic construct
GGYGDDTFL

SEQ ID NO: 4099 - protein, 9 aa, synthetic construct
GGAGGDRLS

SEQ ID NO: 4100 - protein, 9 aa, synthetic construct
GGTGDDQIH

SEQ ID NO: 4101 - protein, 9 aa, synthetic construct
GGDGADRLA

SEQ ID NO: 4102 - protein, 9 aa, synthetic construct
GGRGNDELQ

SEQ ID NO: 4103 - protein, 9 aa, synthetic construct
GGDGDDSLR

SEQ ID NO: 4104 - protein, 9 aa, synthetic construct
GGAGNDSFI

SEQ ID NO: 4105 - protein, 9 aa, synthetic construct
GGMGDDTLT

SEQ ID NO: 4106 - protein, 9 aa, synthetic construct
GGLGNDSLY

SEQ ID NO: 4107 - protein, 9 aa, synthetic construct
GGSGADTLQ

SEQ ID NO: 4108 - protein, 9 aa, synthetic construct
GGSGADSLV

SEQ ID NO: 4109 - protein, 9 aa, synthetic construct
GGRGSDMLT

SEQ ID NO: 4110 - protein, 9 aa, synthetic construct
GGTGNDFIL

SEQ ID NO: 4111 - protein, 9 aa, synthetic construct
GGAGNDVLG

SEQ ID NO: 4112 - protein, 9 aa, synthetic construct
GGIGNDFLS

SEQ ID NO: 4113 - protein, 9 aa, synthetic construct
GGTGDDTVS

SEQ ID NO: 4114 - protein, 9 aa, synthetic construct
GGIGNDSLT

SEQ ID NO: 4115 - protein, 9 aa, synthetic construct
GGAGNDYLF

SEQ ID NO: 4116 - protein, 9 aa, synthetic construct
GGEGADILT

SEQ ID NO: 4117 - protein, 9 aa, synthetic construct
GGIGHDTMD

SEQ ID NO: 4118 - protein, 9 aa, synthetic construct
GGKGDDTYF

SEQ ID NO: 4119 - protein, 9 aa, synthetic construct
GGLGNDNIG

SEQ ID NO: 4120 - protein, 9 aa, synthetic construct
GGLGRDYLS

SEQ ID NO: 4121 - protein, 9 aa, synthetic construct
GGLGNDRLL

SEQ ID NO: 4122 - protein, 9 aa, synthetic construct
GGEGKDVMR

SEQ ID NO: 4123 - protein, 9 aa, synthetic construct
GGAGNDWLA

SEQ ID NO: 4124 - protein, 9 aa, synthetic construct
GGNGRDTFV

SEQ ID NO: 4125 - protein, 9 aa, synthetic construct
GGLGADRLD

SEQ ID NO: 4126 - protein, 9 aa, synthetic construct
GGAGNDGLN

SEQ ID NO: 4127 - protein, 9 aa, synthetic construct
GGEGTDTIS

SEQ ID NO: 4128 - protein, 9 aa, synthetic construct
GGGGSDTID

SEQ ID NO: 4129 - protein, 9 aa, synthetic construct
GGNGNDSID

SEQ ID NO: 4130 - protein, 9 aa, synthetic construct
GGAGNDVIQ

SEQ ID NO: 4131 - protein, 9 aa, synthetic construct
GGSGDDVLK

SEQ ID NO: 4132 - protein, 9 aa, synthetic construct
GGTGNDRIS

SEQ ID NO: 4133 - protein, 9 aa, synthetic construct
GGAGIDRLF

SEQ ID NO: 4134 - protein, 9 aa, synthetic construct
GGAGADRLW

SEQ ID NO: 4135 - protein, 9 aa, synthetic construct
GGDGNDIVR

SEQ ID NO: 4136 - protein, 9 aa, synthetic construct
GGEGADTLF

SEQ ID NO: 4137 - protein, 9 aa, synthetic construct
GGDGNDMLD

SEQ ID NO: 4138 - protein, 9 aa, synthetic construct
GGSGEDLLR

SEQ ID NO: 4139 - protein, 9 aa, synthetic construct
GGLGADRLV

SEQ ID NO: 4140 - protein, 9 aa, synthetic construct
GGIGNDTLQ

SEQ ID NO: 4141 - protein, 9 aa, synthetic construct
GGWGNDVLV

SEQ ID NO: 4142 - protein, 9 aa, synthetic construct
GGDGNDRLQ

SEQ ID NO: 4143 - protein, 9 aa, synthetic construct
GGTGADAMI

SEQ ID NO: 4144 - protein, 9 aa, synthetic construct
GGTGNDRID

SEQ ID NO: 4145 - protein, 9 aa, synthetic construct
GGEGDDKLY

SEQ ID NO: 4146 - protein, 9 aa, synthetic construct
GGGGSDTFT

SEQ ID NO: 4147 - protein, 9 aa, synthetic construct
GGYGNDILD

SEQ ID NO: 4148 - protein, 9 aa, synthetic construct
GGAGNDQIQ

SEQ ID NO: 4149 - protein, 9 aa, synthetic construct
GGLGNDTYK

SEQ ID NO: 4150 - protein, 9 aa, synthetic construct
GGDGADSLV

SEQ ID NO: 4151 - protein, 9 aa, synthetic construct
GGSGRDTFK

SEQ ID NO: 4152 - protein, 9 aa, synthetic construct
GGSGDDRIV

SEQ ID NO: 4153 - protein, 9 aa, synthetic construct
GGDGHDTLD

SEQ ID NO: 4154 - protein, 9 aa, synthetic construct
GGFGHDRLN

SEQ ID NO: 4155 - protein, 9 aa, synthetic construct
GGAGNDSMD

SEQ ID NO: 4156 - protein, 9 aa, synthetic construct
GGNGNDSIN

SEQ ID NO: 4157 - protein, 9 aa, synthetic construct
GGKGDDTLL

SEQ ID NO: 4158 - protein, 9 aa, synthetic construct
GGDGHDTLY

SEQ ID NO: 4159 - protein, 9 aa, synthetic construct
GGFGADTLT

SEQ ID NO: 4160 - protein, 9 aa, synthetic construct
GGDGNDKLV

SEQ ID NO: 4161 - protein, 9 aa, synthetic construct
GGTGNDYLM

SEQ ID NO: 4162 - protein, 9 aa, synthetic construct
GGAGNDSVT

SEQ ID NO: 4163 - protein, 9 aa, synthetic construct
GGSGRDTLD

SEQ ID NO: 4164 - protein, 9 aa, synthetic construct
GGLGSDTFK

SEQ ID NO: 4165 - protein, 9 aa, synthetic construct
GGAGKDTFK

SEQ ID NO: 4166 - protein, 9 aa, synthetic construct
GGIGNDILD

SEQ ID NO: 4167 - protein, 9 aa, synthetic construct
GGAGNDRML

SEQ ID NO: 4168 - protein, 9 aa, synthetic construct
GGAGADKFI

SEQ ID NO: 4169 - protein, 9 aa, synthetic construct
GGGGDDTFR

SEQ ID NO: 4170 - protein, 9 aa, synthetic construct
GGDGNDLII

SEQ ID NO: 4171 - protein, 9 aa, synthetic construct
GGDGNDMLW

SEQ ID NO: 4172 - protein, 9 aa, synthetic construct
GGRGSDTLT

SEQ ID NO: 4173 - protein, 9 aa, synthetic construct
GGAGNDTFT

SEQ ID NO: 4174 - protein, 9 aa, synthetic construct
GGDGADQFF

SEQ ID NO: 4175 - protein, 9 aa, synthetic construct
GGEGADTLA

SEQ ID NO: 4176 - protein, 9 aa, synthetic construct
GGIGDDSLY

SEQ ID NO: 4177 - protein, 9 aa, synthetic construct
GGSGNDALS

SEQ ID NO: 4178 - protein, 9 aa, synthetic construct
GGDGNDVIH

SEQ ID NO: 4179 - protein, 9 aa, synthetic construct
GGEGDDTLH

SEQ ID NO: 4180 - protein, 9 aa, synthetic construct
GGTGDDYMS

SEQ ID NO: 4181 - protein, 9 aa, synthetic construct
GGSGADLLS

SEQ ID NO: 4182 - protein, 9 aa, synthetic construct
GGWGSDLMK

SEQ ID NO: 4183 - protein, 9 aa, synthetic construct
GGGGNDVLH

SEQ ID NO: 4184 - protein, 9 aa, synthetic construct
GGAGNDSYA

SEQ ID NO: 4185 - protein, 9 aa, synthetic construct
GGTGNDLFV

SEQ ID NO: 4186 - protein, 9 aa, synthetic construct
GGLGNDTII

SEQ ID NO: 4187 - protein, 9 aa, synthetic construct
GGDGNDFMG

SEQ ID NO: 4188 - protein, 9 aa, synthetic construct
GGTGNDTAD

SEQ ID NO: 4189 - protein, 9 aa, synthetic construct
GGTGADLLD

SEQ ID NO: 4190 - protein, 9 aa, synthetic construct
GGGGQDQLW

SEQ ID NO: 4191 - protein, 9 aa, synthetic construct
GGSGDDLLN

SEQ ID NO: 4192 - protein, 9 aa, synthetic construct
GGLGNDKLS

SEQ ID NO: 4193 - protein, 9 aa, synthetic construct
GGTGNDLLA

SEQ ID NO: 4194 - protein, 9 aa, synthetic construct
GGAGNDTFF

SEQ ID NO: 4195 - protein, 9 aa, synthetic construct
GGRGNDTLY

SEQ ID NO: 4196 - protein, 9 aa, synthetic construct
GGSGADILD

SEQ ID NO: 4197 - protein, 9 aa, synthetic construct
GGDGSDILV

SEQ ID NO: 4198 - protein, 9 aa, synthetic construct
GGEGVDTLE

SEQ ID NO: 4199 - protein, 9 aa, synthetic construct
GGSGDDALF

SEQ ID NO: 4200 - protein, 9 aa, synthetic construct
GGAGADRMY

SEQ ID NO: 4201 - protein, 9 aa, synthetic construct
GGSGRDVFV

SEQ ID NO: 4202 - protein, 9 aa, synthetic construct
GGDGNDLVN

SEQ ID NO: 4203 - protein, 9 aa, synthetic construct
GGGGNDKLY

SEQ ID NO: 4204 - protein, 9 aa, synthetic construct
GGIGSDTLT

SEQ ID NO: 4205 - protein, 9 aa, synthetic construct
GGDGNDSLE

SEQ ID NO: 4206 - protein, 9 aa, synthetic construct
GGRGSDTLY

SEQ ID NO: 4207 - protein, 9 aa, synthetic construct
GGTGKDTLT

SEQ ID NO: 4208 - protein, 9 aa, synthetic construct
GGSGNDELK

SEQ ID NO: 4209 - protein, 9 aa, synthetic construct
GGYGADQYA

SEQ ID NO: 4210 - protein, 9 aa, synthetic construct
GGAGADHLI

SEQ ID NO: 4211 - protein, 9 aa, synthetic construct
GGTGDDVFV

SEQ ID NO: 4212 - protein, 9 aa, synthetic construct
GGDGADILY

SEQ ID NO: 4213 - protein, 9 aa, synthetic construct
GGAGQDTLV

SEQ ID NO: 4214 - protein, 9 aa, synthetic construct
GGAGNDAVH

SEQ ID NO: 4215 - protein, 9 aa, synthetic construct
GGRGNDRLY

SEQ ID NO: 4216 - protein, 9 aa, synthetic construct
GGSGDDILR

SEQ ID NO: 4217 - protein, 9 aa, synthetic construct
GGFGNDTLS

SEQ ID NO: 4218 - protein, 9 aa, synthetic construct
GGWGNDRLF

SEQ ID NO: 4219 - protein, 9 aa, synthetic construct
GGTGADSLD

SEQ ID NO: 4220 - protein, 9 aa, synthetic construct
GGTGNDWLA

SEQ ID NO: 4221 - protein, 9 aa, synthetic construct
GGSGNDYLV

SEQ ID NO: 4222 - protein, 9 aa, synthetic construct
GGGGNDVYV

SEQ ID NO: 4223 - protein, 9 aa, synthetic construct
GGSGADELR

SEQ ID NO: 4224 - protein, 9 aa, synthetic construct
GGGGNDLIR

SEQ ID NO: 4225 - protein, 9 aa, synthetic construct
GGTGNDIYI

SEQ ID NO: 4226 - protein, 9 aa, synthetic construct
GGKGDDILY

SEQ ID NO: 4227 - protein, 9 aa, synthetic construct
GGDGNDSIN

SEQ ID NO: 4228 - protein, 9 aa, synthetic construct
GGSGRDVLD

SEQ ID NO: 4229 - protein, 9 aa, synthetic construct
GGNGDDRLF

SEQ ID NO: 4230 - protein, 9 aa, synthetic construct
GGTGADMMI

SEQ ID NO: 4231 - protein, 9 aa, synthetic construct
GGTGADILS

SEQ ID NO: 4232 - protein, 9 aa, synthetic construct
GGAGYDYLY

SEQ ID NO: 4233 - protein, 9 aa, synthetic construct
GGEGDDQLA

SEQ ID NO: 4234 - protein, 9 aa, synthetic construct
GGSGNDALN

SEQ ID NO: 4235 - protein, 9 aa, synthetic construct
GGGGSDTML

SEQ ID NO: 4236 - protein, 9 aa, synthetic construct
GGAGADELR

SEQ ID NO: 4237 - protein, 9 aa, synthetic construct
GGDGNDFLD

SEQ ID NO: 4238 - protein, 9 aa, synthetic construct
GGAGNDAIS

SEQ ID NO: 4239 - protein, 9 aa, synthetic construct
GGKGDDSLS

SEQ ID NO: 4240 - protein, 9 aa, synthetic construct
GGSGDDVIS

SEQ ID NO: 4241 - protein, 9 aa, synthetic construct
GGAGADRFA

SEQ ID NO: 4242 - protein, 9 aa, synthetic construct
GGSGADQLT

SEQ ID NO: 4243 - protein, 9 aa, synthetic construct
GGIGDDTIY

SEQ ID NO: 4244 - protein, 9 aa, synthetic construct
GGEGADSLD

SEQ ID NO: 4245 - protein, 9 aa, synthetic construct
GGSGADVLI

SEQ ID NO: 4246 - protein, 9 aa, synthetic construct
GGDGADLFV

SEQ ID NO: 4247 - protein, 9 aa, synthetic construct
GGKGDDLLI

SEQ ID NO: 4248 - protein, 9 aa, synthetic construct
GGDGNDSMV

SEQ ID NO: 4249 - protein, 9 aa, synthetic construct
GGSGDDTFV

SEQ ID NO: 4250 - protein, 9 aa, synthetic construct
GGTGDDYLE

SEQ ID NO: 4251 - protein, 9 aa, synthetic construct
GGTGNDSLF

SEQ ID NO: 4252 - protein, 9 aa, synthetic construct
GGTGNDTYT

SEQ ID NO: 4253 - protein, 9 aa, synthetic construct
GGDGDDWLE

SEQ ID NO: 4254 - protein, 9 aa, synthetic construct
GGDGDDTVF

SEQ ID NO: 4255 - protein, 9 aa, synthetic construct
GGLGADVLN

SEQ ID NO: 4256 - protein, 9 aa, synthetic construct
GGAGADVMS

SEQ ID NO: 4257 - protein, 9 aa, synthetic construct
GGNGDDTLT

SEQ ID NO: 4258 - protein, 9 aa, synthetic construct
GGAGDDIII

SEQ ID NO: 4259 - protein, 9 aa, synthetic construct
GGDGNDAID

SEQ ID NO: 4260 - protein, 9 aa, synthetic construct
GGAGHDTLS

SEQ ID NO: 4261 - protein, 9 aa, synthetic construct
GGKGNDLLQ

SEQ ID NO: 4262 - protein, 9 aa, synthetic construct
GGVGRDVIF

SEQ ID NO: 4263 - protein, 9 aa, synthetic construct
GGAGDDQID

SEQ ID NO: 4264 - protein, 9 aa, synthetic construct
GGRGDDVLI

SEQ ID NO: 4265 - protein, 9 aa, synthetic construct
GGSGGDTLV

SEQ ID NO: 4266 - protein, 9 aa, synthetic construct
GGRGADTLN

SEQ ID NO: 4267 - protein, 9 aa, synthetic construct
GGGGEDVFV

SEQ ID NO: 4268 - protein, 9 aa, synthetic construct
GGAGDDLMR

SEQ ID NO: 4269 - protein, 9 aa, synthetic construct
GGGGNDTMT

SEQ ID NO: 4270 - protein, 9 aa, synthetic construct
GGLGADVLS

SEQ ID NO: 4271 - protein, 9 aa, synthetic construct
GGAGADTFD

SEQ ID NO: 4272 - protein, 9 aa, synthetic construct
GGWGDDTFH

SEQ ID NO: 4273 - protein, 9 aa, synthetic construct
GGRGDDTYV

SEQ ID NO: 4274 - protein, 9 aa, synthetic construct
GGAGDDIIR

SEQ ID NO: 4275 - protein, 9 aa, synthetic construct
GGGGADQLH

SEQ ID NO: 4276 - protein, 9 aa, synthetic construct
GGVGHDYLY

SEQ ID NO: 4277 - protein, 9 aa, synthetic construct
GGKGDDVLF

SEQ ID NO: 4278 - protein, 9 aa, synthetic construct
GGAGDDAYL

SEQ ID NO: 4279 - protein, 9 aa, synthetic construct
GGAGVDTLN

SEQ ID NO: 4280 - protein, 9 aa, synthetic construct
GGNGNDTLQ

SEQ ID NO: 4281 - protein, 9 aa, synthetic construct
GGLGDDFLS

SEQ ID NO: 4282 - protein, 9 aa, synthetic construct
GGEGSDTFV

SEQ ID NO: 4283 - protein, 9 aa, synthetic construct
GGEGDDILF

SEQ ID NO: 4284 - protein, 9 aa, synthetic construct
GGAGDDVII

SEQ ID NO: 4285 - protein, 9 aa, synthetic construct
GGEGNDVLR

SEQ ID NO: 4286 - protein, 9 aa, synthetic construct
GGAGTDTIN

SEQ ID NO: 4287 - protein, 9 aa, synthetic construct
GGTGADVMI

SEQ ID NO: 4288 - protein, 9 aa, synthetic construct
GGNGLDTAS

SEQ ID NO: 4289 - protein, 9 aa, synthetic construct
GGEGSDTYL

SEQ ID NO: 4290 - protein, 9 aa, synthetic construct
GGEGDDAVY

SEQ ID NO: 4291 - protein, 9 aa, synthetic construct
GGLGDDTIF

SEQ ID NO: 4292 - protein, 9 aa, synthetic construct
GGLGDDTIL

SEQ ID NO: 4293 - protein, 9 aa, synthetic construct
GGVGNDSLY

SEQ ID NO: 4294 - protein, 9 aa, synthetic construct
GGTGDDMLF

SEQ ID NO: 4295 - protein, 9 aa, synthetic construct
GGAGSDVLR

SEQ ID NO: 4296 - protein, 9 aa, synthetic construct
GGRGEDRMI

SEQ ID NO: 4297 - protein, 9 aa, synthetic construct
GGAGRDKLS

SEQ ID NO: 4298 - protein, 9 aa, synthetic construct
GGVGRDTLV

SEQ ID NO: 4299 - protein, 9 aa, synthetic construct
GGSGHDTLD

SEQ ID NO: 4300 - protein, 9 aa, synthetic construct
GGGGIDTLS

SEQ ID NO: 4301 - protein, 9 aa, synthetic construct
GGAGDDHLL

SEQ ID NO: 4302 - protein, 9 aa, synthetic construct
GGEGDDVLS

SEQ ID NO: 4303 - protein, 9 aa, synthetic construct
GGIGNDYLY

SEQ ID NO: 4304 - protein, 9 aa, synthetic construct
GGAGIDTVS

SEQ ID NO: 4305 - protein, 9 aa, synthetic construct
GGQGNDIMT

SEQ ID NO: 4306 - protein, 9 aa, synthetic construct
GGDGHDVLH

SEQ ID NO: 4307 - protein, 9 aa, synthetic construct
GGAGDDHLY

SEQ ID NO: 4308 - protein, 9 aa, synthetic construct
GGAGDDTVS

SEQ ID NO: 4309 - protein, 9 aa, synthetic construct
GGAGDDTVT

SEQ ID NO: 4310 - protein, 9 aa, synthetic construct
GGDGDDTIR

SEQ ID NO: 4311 - protein, 9 aa, synthetic construct
GGSGNDTYQ

SEQ ID NO: 4312 - protein, 9 aa, synthetic construct
GGAGRDTLF

SEQ ID NO: 4313 - protein, 9 aa, synthetic construct
GGSGHDTLY

SEQ ID NO: 4314 - protein, 9 aa, synthetic construct
GGDGNDTFI

SEQ ID NO: 4315 - protein, 9 aa, synthetic construct
GGDGVDTLI

SEQ ID NO: 4316 - protein, 9 aa, synthetic construct
GGLGADVLI

SEQ ID NO: 4317 - protein, 9 aa, synthetic construct
GGFGRDRLT

SEQ ID NO: 4318 - protein, 9 aa, synthetic construct
GGGGNDSLT

SEQ ID NO: 4319 - protein, 9 aa, synthetic construct
GGSGHDLLR

SEQ ID NO: 4320 - protein, 9 aa, synthetic construct
GGEGDDLLL

SEQ ID NO: 4321 - protein, 9 aa, synthetic construct
GGMGNDTLL

SEQ ID NO: 4322 - protein, 9 aa, synthetic construct
GGGGNDVIA

SEQ ID NO: 4323 - protein, 9 aa, synthetic construct
GGAGDDILK

SEQ ID NO: 4324 - protein, 9 aa, synthetic construct
GGVGNDVLS

SEQ ID NO: 4325 - protein, 9 aa, synthetic construct
GGIGADHLW

SEQ ID NO: 4326 - protein, 9 aa, synthetic construct
GGTGSDRLV

SEQ ID NO: 4327 - protein, 9 aa, synthetic construct
GGLGNDALY

SEQ ID NO: 4328 - protein, 9 aa, synthetic construct
GGAGKDILT

SEQ ID NO: 4329 - protein, 9 aa, synthetic construct
GGGGLDRLR

SEQ ID NO: 4330 - protein, 9 aa, synthetic construct
GGTGDDLLF

SEQ ID NO: 4331 - protein, 9 aa, synthetic construct
GGNGNDILF

SEQ ID NO: 4332 - protein, 9 aa, synthetic construct
GGTGSDILT

SEQ ID NO: 4333 - protein, 9 aa, synthetic construct
GGKGNDIYF

SEQ ID NO: 4334 - protein, 9 aa, synthetic construct
GGAGSDIYI

SEQ ID NO: 4335 - protein, 9 aa, synthetic construct
GGLGTDTLD

SEQ ID NO: 4336 - protein, 9 aa, synthetic construct
GGLGDDVYL

SEQ ID NO: 4337 - protein, 9 aa, synthetic construct
GGSGSDRYI

SEQ ID NO: 4338 - protein, 9 aa, synthetic construct
GGQGHDTLI

SEQ ID NO: 4339 - protein, 9 aa, synthetic construct
GGDGSDTID

SEQ ID NO: 4340 - protein, 9 aa, synthetic construct
GGGGADSIT

SEQ ID NO: 4341 - protein, 9 aa, synthetic construct
GGSGNDIIY

SEQ ID NO: 4342 - protein, 9 aa, synthetic construct
GGEGDDEII

SEQ ID NO: 4343 - protein, 9 aa, synthetic construct
GGTGSDKLN

SEQ ID NO: 4344 - protein, 9 aa, synthetic construct
GGAGDDQLH

SEQ ID NO: 4345 - protein, 9 aa, synthetic construct
GGDGNDTIE

SEQ ID NO: 4346 - protein, 9 aa, synthetic construct
GGDGTDLLV

SEQ ID NO: 4347 - protein, 9 aa, synthetic construct
GGIGADTLD

SEQ ID NO: 4348 - protein, 9 aa, synthetic construct
GGTGDDLLY

SEQ ID NO: 4349 - protein, 9 aa, synthetic construct
GGSGNDTVT

SEQ ID NO: 4350 - protein, 9 aa, synthetic construct
GGGGADVLK

SEQ ID NO: 4351 - protein, 9 aa, synthetic construct
GGDGDDTLQ

SEQ ID NO: 4352 - protein, 9 aa, synthetic construct
GGSGNDQFR

SEQ ID NO: 4353 - protein, 9 aa, synthetic construct
GGRGDDLLI

SEQ ID NO: 4354 - protein, 9 aa, synthetic construct
GGNGDDKLY

SEQ ID NO: 4355 - protein, 9 aa, synthetic construct
GGTGADTIN

SEQ ID NO: 4356 - protein, 9 aa, synthetic construct
GGDGSDYLT

SEQ ID NO: 4357 - protein, 9 aa, synthetic construct
GGDGSDTLN

SEQ ID NO: 4358 - protein, 9 aa, synthetic construct
GGDGDDTLG

SEQ ID NO: 4359 - protein, 9 aa, synthetic construct
GGVGNDTLA

SEQ ID NO: 4360 - protein, 9 aa, synthetic construct
GGAGSDTYY

SEQ ID NO: 4361 - protein, 9 aa, synthetic construct
GGAGDDLLH

SEQ ID NO: 4362 - protein, 9 aa, synthetic construct
GGAGHDTLY

SEQ ID NO: 4363 - protein, 9 aa, synthetic construct
GGSGTDTLV

SEQ ID NO: 4364 - protein, 9 aa, synthetic construct
GGTGSDTLF

SEQ ID NO: 4365 - protein, 9 aa, synthetic construct
GGKGNDLLT

SEQ ID NO: 4366 - protein, 9 aa, synthetic construct
GGDGGDTFI

SEQ ID NO: 4367 - protein, 9 aa, synthetic construct
GGAGDDSIS

SEQ ID NO: 4368 - protein, 9 aa, synthetic construct
GGNGNDFLY

SEQ ID NO: 4369 - protein, 9 aa, synthetic construct
GGDGPDHLI

SEQ ID NO: 4370 - protein, 9 aa, synthetic construct
GGDGDDKLF

SEQ ID NO: 4371 - protein, 9 aa, synthetic construct
GGAGNDLMS

SEQ ID NO: 4372 - protein, 9 aa, synthetic construct
GGAGRDSLN

SEQ ID NO: 4373 - protein, 9 aa, synthetic construct
GGFGNDLLN

SEQ ID NO: 4374 - protein, 9 aa, synthetic construct
GGAGNDIYH

SEQ ID NO: 4375 - protein, 9 aa, synthetic construct
GGAGHDVLE

SEQ ID NO: 4376 - protein, 9 aa, synthetic construct
GGAGADVMT

SEQ ID NO: 4377 - protein, 9 aa, synthetic construct
GGNGNDILK

SEQ ID NO: 4378 - protein, 9 aa, synthetic construct
GGPGTDTLT

SEQ ID NO: 4379 - protein, 9 aa, synthetic construct
GGNGDDMLT

SEQ ID NO: 4380 - protein, 9 aa, synthetic construct
GGDGNDTIW

SEQ ID NO: 4381 - protein, 9 aa, synthetic construct
GGGGNDTVS

SEQ ID NO: 4382 - protein, 9 aa, synthetic construct
GGGGDDLLN

SEQ ID NO: 4383 - protein, 9 aa, synthetic construct
GGDGNDALI

SEQ ID NO: 4384 - protein, 9 aa, synthetic construct
GGQGQDLLD

SEQ ID NO: 4385 - protein, 9 aa, synthetic construct
GGGGADMFI

SEQ ID NO: 4386 - protein, 9 aa, synthetic construct
GGAGNDIYL

SEQ ID NO: 4387 - protein, 9 aa, synthetic construct
GGEGNDVLN

SEQ ID NO: 4388 - protein, 9 aa, synthetic construct
GGAGADTMQ

SEQ ID NO: 4389 - protein, 9 aa, synthetic construct
GGAGDDAIS

SEQ ID NO: 4390 - protein, 9 aa, synthetic construct
GGVGADRLE

SEQ ID NO: 4391 - protein, 9 aa, synthetic construct
GGKGDDTYW

SEQ ID NO: 4392 - protein, 9 aa, synthetic construct
GGDGVDRVV

SEQ ID NO: 4393 - protein, 9 aa, synthetic construct
GGQGDDILN

SEQ ID NO: 4394 - protein, 9 aa, synthetic construct
GGNGNDVIS

SEQ ID NO: 4395 - protein, 9 aa, synthetic construct
GGEGNDSLI

SEQ ID NO: 4396 - protein, 9 aa, synthetic construct
GGSGNDTFL

SEQ ID NO: 4397 - protein, 9 aa, synthetic construct
GGAGDDTFI

SEQ ID NO: 4398 - protein, 9 aa, synthetic construct
GGTGRDHIY

SEQ ID NO: 4399 - protein, 9 aa, synthetic construct
GGLGIDTLV

SEQ ID NO: 4400 - protein, 9 aa, synthetic construct
GGDGKDTFK

SEQ ID NO: 4401 - protein, 9 aa, synthetic construct
GGAGKDMLK

SEQ ID NO: 4402 - protein, 9 aa, synthetic construct
GGAGKDAFV

SEQ ID NO: 4403 - protein, 9 aa, synthetic construct
GGGGADQLY

SEQ ID NO: 4404 - protein, 9 aa, synthetic construct
GGPGRDLLD

SEQ ID NO: 4405 - protein, 9 aa, synthetic construct
GGRGADLLD

SEQ ID NO: 4406 - protein, 9 aa, synthetic construct
GGQGADTLR

SEQ ID NO: 4407 - protein, 9 aa, synthetic construct
GGGGIDSLT

SEQ ID NO: 4408 - protein, 9 aa, synthetic construct
GGDGMDFIN

SEQ ID NO: 4409 - protein, 9 aa, synthetic construct
GGEGNDELN

SEQ ID NO: 4410 - protein, 9 aa, synthetic construct
GGNGDDQLT

SEQ ID NO: 4411 - protein, 9 aa, synthetic construct
GGDGNDELH

SEQ ID NO: 4412 - protein, 9 aa, synthetic construct
GGSGNDTIV

SEQ ID NO: 4413 - protein, 9 aa, synthetic construct
GGDGDDTIG

SEQ ID NO: 4414 - protein, 9 aa, synthetic construct
GGAGRDVLH

SEQ ID NO: 4415 - protein, 9 aa, synthetic construct
GGVGNDIVN

SEQ ID NO: 4416 - protein, 9 aa, synthetic construct
GGSGNDVIE

SEQ ID NO: 4417 - protein, 9 aa, synthetic construct
GGLGDDLVN

SEQ ID NO: 4418 - protein, 9 aa, synthetic construct
GGQGSDSIR

SEQ ID NO: 4419 - protein, 9 aa, synthetic construct
GGAGDDFLR

SEQ ID NO: 4420 - protein, 9 aa, synthetic construct
GGVGNDHLY

SEQ ID NO: 4421 - protein, 9 aa, synthetic construct
GGAGDDFLI

SEQ ID NO: 4422 - protein, 9 aa, synthetic construct
GGLGDDIYL

SEQ ID NO: 4423 - protein, 9 aa, synthetic construct
GGNGADILD

SEQ ID NO: 4424 - protein, 9 aa, synthetic construct
GGNGNDAIV

SEQ ID NO: 4425 - protein, 9 aa, synthetic construct
GGEGGDYVA

SEQ ID NO: 4426 - protein, 9 aa, synthetic construct
GGMGLDTLD

SEQ ID NO: 4427 - protein, 9 aa, synthetic construct
GGSGNDLIT

SEQ ID NO: 4428 - protein, 9 aa, synthetic construct
GGSGNDTLM

SEQ ID NO: 4429 - protein, 9 aa, synthetic construct
GGEGDDHLI

SEQ ID NO: 4430 - protein, 9 aa, synthetic construct
GGTGTDRLT

SEQ ID NO: 4431 - protein, 9 aa, synthetic construct
GGAGRDHLE

SEQ ID NO: 4432 - protein, 9 aa, synthetic construct
GGEGNDSLS

SEQ ID NO: 4433 - protein, 9 aa, synthetic construct
GGRGADDLN

SEQ ID NO: 4434 - protein, 9 aa, synthetic construct
GGDGNDYIE

SEQ ID NO: 4435 - protein, 9 aa, synthetic construct
GGSGNDLIR

SEQ ID NO: 4436 - protein, 9 aa, synthetic construct
GGHGEDILN

SEQ ID NO: 4437 - protein, 9 aa, synthetic construct
GGDGDDVIR

SEQ ID NO: 4438 - protein, 9 aa, synthetic construct
GGAGHDSLV

SEQ ID NO: 4439 - protein, 9 aa, synthetic construct
GGTGTDTAV

SEQ ID NO: 4440 - protein, 9 aa, synthetic construct
GGDGDDTYD

SEQ ID NO: 4441 - protein, 9 aa, synthetic construct
GGKGNDAYA

SEQ ID NO: 4442 - protein, 9 aa, synthetic construct
GGDGNDTAS

SEQ ID NO: 4443 - protein, 9 aa, synthetic construct
GGAGRDVLD

SEQ ID NO: 4444 - protein, 9 aa, synthetic construct
GGAGNDIIW

SEQ ID NO: 4445 - protein, 9 aa, synthetic construct
GGEGDDVLN

SEQ ID NO: 4446 - protein, 9 aa, synthetic construct
GGDGNDQLT

SEQ ID NO: 4447 - protein, 9 aa, synthetic construct
GGNGNDVIN

SEQ ID NO: 4448 - protein, 9 aa, synthetic construct
GGLGRDALY

SEQ ID NO: 4449 - protein, 9 aa, synthetic construct
GGGGDDRIF

SEQ ID NO: 4450 - protein, 9 aa, synthetic construct
GGGGADRYL

SEQ ID NO: 4451 - protein, 9 aa, synthetic construct
GGVGTDSLS

SEQ ID NO: 4452 - protein, 9 aa, synthetic construct
GGQGNDLLD

SEQ ID NO: 4453 - protein, 9 aa, synthetic construct
GGNGNDELY

SEQ ID NO: 4454 - protein, 9 aa, synthetic construct
GGDGNDEID

SEQ ID NO: 4455 - protein, 9 aa, synthetic construct
GGAGNDLIR

SEQ ID NO: 4456 - protein, 9 aa, synthetic construct
GGEGNDILE

SEQ ID NO: 4457 - protein, 9 aa, synthetic construct
GGVGDDIYI

SEQ ID NO: 4458 - protein, 9 aa, synthetic construct
GGNGNDALD

SEQ ID NO: 4459 - protein, 9 aa, synthetic construct
GGGGADSLV

SEQ ID NO: 4460 - protein, 9 aa, synthetic construct
GGAGRDTMT

SEQ ID NO: 4461 - protein, 9 aa, synthetic construct
GGDGDDFLF

SEQ ID NO: 4462 - protein, 9 aa, synthetic construct
GGKGDDWLD

SEQ ID NO: 4463 - protein, 9 aa, synthetic construct
GGDGTDTLS

SEQ ID NO: 4464 - protein, 9 aa, synthetic construct
GGPGNDLLR

SEQ ID NO: 4465 - protein, 9 aa, synthetic construct
GGAGDDNLY

SEQ ID NO: 4466 - protein, 9 aa, synthetic construct
GGGGADLFV

SEQ ID NO: 4467 - protein, 9 aa, synthetic construct
GGEGADLLL

SEQ ID NO: 4468 - protein, 9 aa, synthetic construct
GGDGSDTYI

SEQ ID NO: 4469 - protein, 9 aa, synthetic construct
GGVGDDTLL

SEQ ID NO: 4470 - protein, 9 aa, synthetic construct
GGAGADTMK

SEQ ID NO: 4471 - protein, 9 aa, synthetic construct
GGAGADTMF

SEQ ID NO: 4472 - protein, 9 aa, synthetic construct
GGTGNDLLR

SEQ ID NO: 4473 - protein, 9 aa, synthetic construct
GGEGKDTVR

SEQ ID NO: 4474 - protein, 9 aa, synthetic construct
GGAGNDTVF

SEQ ID NO: 4475 - protein, 9 aa, synthetic construct
GGSGNDTVY

SEQ ID NO: 4476 - protein, 9 aa, synthetic construct
GGSGHDTIL

SEQ ID NO: 4477 - protein, 9 aa, synthetic construct
GGGGNDTFR

SEQ ID NO: 4478 - protein, 9 aa, synthetic construct
GGDGGDYLA

SEQ ID NO: 4479 - protein, 9 aa, synthetic construct
GGAGDDSVS

SEQ ID NO: 4480 - protein, 9 aa, synthetic construct
GGHGNDTLD

SEQ ID NO: 4481 - protein, 9 aa, synthetic construct
GGNGNDSLS

SEQ ID NO: 4482 - protein, 9 aa, synthetic construct
GGDGNDALN

SEQ ID NO: 4483 - protein, 9 aa, synthetic construct
GGSGADRME

SEQ ID NO: 4484 - protein, 9 aa, synthetic construct
GGAGGDLLS

SEQ ID NO: 4485 - protein, 9 aa, synthetic construct
GGSGADVLR

SEQ ID NO: 4486 - protein, 9 aa, synthetic construct
GGLGHDYMD

SEQ ID NO: 4487 - protein, 9 aa, synthetic construct
GGAGGDLME

SEQ ID NO: 4488 - protein, 9 aa, synthetic construct
GGAGRDVFI

SEQ ID NO: 4489 - protein, 9 aa, synthetic construct
GGAGNDTFS

SEQ ID NO: 4490 - protein, 9 aa, synthetic construct
GGAGSDRYE

SEQ ID NO: 4491 - protein, 9 aa, synthetic construct
GGEGRDTLN

SEQ ID NO: 4492 - protein, 9 aa, synthetic construct
GGKGDDTLD

SEQ ID NO: 4493 - protein, 9 aa, synthetic construct
GGAGDDTIH

SEQ ID NO: 4494 - protein, 9 aa, synthetic construct
GGKGDDILV

SEQ ID NO: 4495 - protein, 9 aa, synthetic construct
GGAGDDQLA

SEQ ID NO: 4496 - protein, 9 aa, synthetic construct
GGGGADEIR

SEQ ID NO: 4497 - protein, 9 aa, synthetic construct
GGAGNDTVW

SEQ ID NO: 4498 - protein, 9 aa, synthetic construct
GGQGNDSIV

SEQ ID NO: 4499 - protein, 9 aa, synthetic construct
GGIGNDILN

SEQ ID NO: 4500 - protein, 9 aa, synthetic construct
GGTGDDVID

SEQ ID NO: 4501 - protein, 9 aa, synthetic construct
GGNGDDALA

SEQ ID NO: 4502 - protein, 9 aa, synthetic construct
GGFGNDVLN

SEQ ID NO: 4503 - protein, 9 aa, synthetic construct
GGNGIDTAS

SEQ ID NO: 4504 - protein, 9 aa, synthetic construct
GGAGRDRLA

SEQ ID NO: 4505 - protein, 9 aa, synthetic construct
GGTGHDTLY

SEQ ID NO: 4506 - protein, 9 aa, synthetic construct
GGVGNDVLQ

SEQ ID NO: 4507 - protein, 9 aa, synthetic construct
GGAGRDRFV

SEQ ID NO: 4508 - protein, 9 aa, synthetic construct
GGDGNDSMY

SEQ ID NO: 4509 - protein, 9 aa, synthetic construct
GGTGNDLID

SEQ ID NO: 4510 - protein, 9 aa, synthetic construct
GGNGDDSLI

SEQ ID NO: 4511 - protein, 9 aa, synthetic construct
GGSGNDLLK

SEQ ID NO: 4512 - protein, 9 aa, synthetic construct
GGAGNDSYY

SEQ ID NO: 4513 - protein, 9 aa, synthetic construct
GGRGDDLLD

SEQ ID NO: 4514 - protein, 9 aa, synthetic construct
GGSGDDVIY

SEQ ID NO: 4515 - protein, 9 aa, synthetic construct
GGAGDDVVR

SEQ ID NO: 4516 - protein, 9 aa, synthetic construct
GGAGADAMA

SEQ ID NO: 4517 - protein, 9 aa, synthetic construct
GGSGDDTIE

SEQ ID NO: 4518 - protein, 9 aa, synthetic construct
GGTGHDTLD

SEQ ID NO: 4519 - protein, 9 aa, synthetic construct
GGDGSDTYY

SEQ ID NO: 4520 - protein, 9 aa, synthetic construct
GGKGDDVLH

SEQ ID NO: 4521 - protein, 9 aa, synthetic construct
GGSGADLLV

SEQ ID NO: 4522 - protein, 9 aa, synthetic construct
GGLGDDLID

SEQ ID NO: 4523 - protein, 9 aa, synthetic construct
GGAGNDIVT

SEQ ID NO: 4524 - protein, 9 aa, synthetic construct
GGLGNDSLA

SEQ ID NO: 4525 - protein, 9 aa, synthetic construct
GGGGDDLLY

SEQ ID NO: 4526 - protein, 9 aa, synthetic construct
GGTGNDSIH

SEQ ID NO: 4527 - protein, 9 aa, synthetic construct
GGMGSDTLT

SEQ ID NO: 4528 - protein, 9 aa, synthetic construct
GGAGADLLQ

SEQ ID NO: 4529 - protein, 9 aa, synthetic construct
GGDGRDVLY

SEQ ID NO: 4530 - protein, 9 aa, synthetic construct
GGGGNDSLL

SEQ ID NO: 4531 - protein, 9 aa, synthetic construct
GGWGADTLI

SEQ ID NO: 4532 - protein, 9 aa, synthetic construct
GGKGNDILY

SEQ ID NO: 4533 - protein, 9 aa, synthetic construct
GGDGNDILH

SEQ ID NO: 4534 - protein, 9 aa, synthetic construct
GGAGDDNLD

SEQ ID NO: 4535 - protein, 9 aa, synthetic construct
GGGGADRLF

SEQ ID NO: 4536 - protein, 9 aa, synthetic construct
GGDGNDTVT

SEQ ID NO: 4537 - protein, 9 aa, synthetic construct
GGDGNDQLI

SEQ ID NO: 4538 - protein, 9 aa, synthetic construct
GGTGNDSIY

SEQ ID NO: 4539 - protein, 9 aa, synthetic construct
GGVGDDVLE

SEQ ID NO: 4540 - protein, 9 aa, synthetic construct
GGLGNDALF

SEQ ID NO: 4541 - protein, 9 aa, synthetic construct
GGLGNDKLV

SEQ ID NO: 4542 - protein, 9 aa, synthetic construct
GGGGADVLD

SEQ ID NO: 4543 - protein, 9 aa, synthetic construct
GGAGDDVMD

SEQ ID NO: 4544 - protein, 9 aa, synthetic construct
GGRGDDIFV

SEQ ID NO: 4545 - protein, 9 aa, synthetic construct
GGTGDDVMT

SEQ ID NO: 4546 - protein, 9 aa, synthetic construct
GGDGRDTYV

SEQ ID NO: 4547 - protein, 9 aa, synthetic construct
GGSGGDVLN

SEQ ID NO: 4548 - protein, 9 aa, synthetic construct
GGQGNDILL

SEQ ID NO: 4549 - protein, 9 aa, synthetic construct
GGDGADHLA

SEQ ID NO: 4550 - protein, 9 aa, synthetic construct
GGEGADTIT

SEQ ID NO: 4551 - protein, 9 aa, synthetic construct
GGEGRDTLF

SEQ ID NO: 4552 - protein, 9 aa, synthetic construct
GGDGNDVAD

SEQ ID NO: 4553 - protein, 9 aa, synthetic construct
GGDGDDELA

SEQ ID NO: 4554 - protein, 9 aa, synthetic construct
GGAGRDTIS

SEQ ID NO: 4555 - protein, 9 aa, synthetic construct
GGTGDDVLH

SEQ ID NO: 4556 - protein, 9 aa, synthetic construct
GGMGDDQLI

SEQ ID NO: 4557 - protein, 9 aa, synthetic construct
GGNGADTLT

SEQ ID NO: 4558 - protein, 9 aa, synthetic construct
GGLGDDTLQ

SEQ ID NO: 4559 - protein, 9 aa, synthetic construct
GGTGDDTYY

SEQ ID NO: 4560 - protein, 9 aa, synthetic construct
GGTGDDTFI

SEQ ID NO: 4561 - protein, 9 aa, synthetic construct
GGAGSDSLF

SEQ ID NO: 4562 - protein, 9 aa, synthetic construct
GGAGADVIV

SEQ ID NO: 4563 - protein, 9 aa, synthetic construct
GGDGEDQLE

SEQ ID NO: 4564 - protein, 9 aa, synthetic construct
GGSGNDRLA

SEQ ID NO: 4565 - protein, 9 aa, synthetic construct
GGDGADTIV

SEQ ID NO: 4566 - protein, 9 aa, synthetic construct
GGAGRDVMR

SEQ ID NO: 4567 - protein, 9 aa, synthetic construct
GGDGDDVLK

SEQ ID NO: 4568 - protein, 9 aa, synthetic construct
GGTGADDLN

SEQ ID NO: 4569 - protein, 9 aa, synthetic construct
GGAGNDVAN

SEQ ID NO: 4570 - protein, 9 aa, synthetic construct
GGEGGDLLV

SEQ ID NO: 4571 - protein, 9 aa, synthetic construct
GGEGNDRLA

SEQ ID NO: 4572 - protein, 9 aa, synthetic construct
GGSGADTLR

SEQ ID NO: 4573 - protein, 9 aa, synthetic construct
GGKGDDMLS

SEQ ID NO: 4574 - protein, 9 aa, synthetic construct
GGAGRDTLR

SEQ ID NO: 4575 - protein, 9 aa, synthetic construct
GGEGNDVLY

SEQ ID NO: 4576 - protein, 9 aa, synthetic construct
GGIGNDDLD

SEQ ID NO: 4577 - protein, 9 aa, synthetic construct
GGEGRDLLD

SEQ ID NO: 4578 - protein, 9 aa, synthetic construct
GGAGRDTLQ

SEQ ID NO: 4579 - protein, 9 aa, synthetic construct
GGAGNDDIN

SEQ ID NO: 4580 - protein, 9 aa, synthetic construct
GGEGADRLE

SEQ ID NO: 4581 - protein, 9 aa, synthetic construct
GGSGADTFK

SEQ ID NO: 4582 - protein, 9 aa, synthetic construct
GGQGNDTLR

SEQ ID NO: 4583 - protein, 9 aa, synthetic construct
GGAGADVMN

SEQ ID NO: 4584 - protein, 9 aa, synthetic construct
GGLGDDTIN

SEQ ID NO: 4585 - protein, 9 aa, synthetic construct
GGDGADVIY

SEQ ID NO: 4586 - protein, 9 aa, synthetic construct
GGDGNDVLG

SEQ ID NO: 4587 - protein, 9 aa, synthetic construct
GGEGNDMLF

SEQ ID NO: 4588 - protein, 9 aa, synthetic construct
GGPGNDNIG

SEQ ID NO: 4589 - protein, 9 aa, synthetic construct
GGMGDDMYV

SEQ ID NO: 4590 - protein, 9 aa, synthetic construct
GGDGIDTIN

SEQ ID NO: 4591 - protein, 9 aa, synthetic construct
GGAGVDNLY

SEQ ID NO: 4592 - protein, 9 aa, synthetic construct
GGIGDDVYV

SEQ ID NO: 4593 - protein, 9 aa, synthetic construct
GGVGDDLLN

SEQ ID NO: 4594 - protein, 9 aa, synthetic construct
GGQGNDILR

SEQ ID NO: 4595 - protein, 9 aa, synthetic construct
GGAGNDQIT

SEQ ID NO: 4596 - protein, 9 aa, synthetic construct
GGVGRDSLY

SEQ ID NO: 4597 - protein, 9 aa, synthetic construct
GGAGRDWLD

SEQ ID NO: 4598 - protein, 9 aa, synthetic construct
GGAGADTVS

SEQ ID NO: 4599 - protein, 9 aa, synthetic construct
GGAGIDQLS

SEQ ID NO: 4600 - protein, 9 aa, synthetic construct
GGAGDDTIW

SEQ ID NO: 4601 - protein, 9 aa, synthetic construct
GGVGDDEIL

SEQ ID NO: 4602 - protein, 9 aa, synthetic construct
GGEGEDTLV

SEQ ID NO: 4603 - protein, 9 aa, synthetic construct
GGAGNDQLA

SEQ ID NO: 4604 - protein, 9 aa, synthetic construct
GGTGDDSVS

SEQ ID NO: 4605 - protein, 9 aa, synthetic construct
GGAGLDTLT

SEQ ID NO: 4606 - protein, 9 aa, synthetic construct
GGAGSDLLR

SEQ ID NO: 4607 - protein, 9 aa, synthetic construct
GGNGADSLY

SEQ ID NO: 4608 - protein, 9 aa, synthetic construct
GGAGKDQFV

SEQ ID NO: 4609 - protein, 9 aa, synthetic construct
GGGGNDRLW

SEQ ID NO: 4610 - protein, 9 aa, synthetic construct
GGLGRDVFK

SEQ ID NO: 4611 - protein, 9 aa, synthetic construct
GGDGADILS

SEQ ID NO: 4612 - protein, 9 aa, synthetic construct
GGKGNDILN

SEQ ID NO: 4613 - protein, 9 aa, synthetic construct
GGKGNDHLT

SEQ ID NO: 4614 - protein, 9 aa, synthetic construct
GGLGDDFIH

SEQ ID NO: 4615 - protein, 9 aa, synthetic construct
GGAGDDLIR

SEQ ID NO: 4616 - protein, 9 aa, synthetic construct
GGGGNDTYY

SEQ ID NO: 4617 - protein, 9 aa, synthetic construct
GGDGDDDLF

SEQ ID NO: 4618 - protein, 9 aa, synthetic construct
GGLGNDNLY

SEQ ID NO: 4619 - protein, 9 aa, synthetic construct
GGEGDDYLH

SEQ ID NO: 4620 - protein, 9 aa, synthetic construct
GGAGSDMLN

SEQ ID NO: 4621 - protein, 9 aa, synthetic construct
GGSGNDRIE

SEQ ID NO: 4622 - protein, 9 aa, synthetic construct
GGEGKDIFV

SEQ ID NO: 4623 - protein, 9 aa, synthetic construct
GGDGNDLLW

SEQ ID NO: 4624 - protein, 9 aa, synthetic construct
GGLGDDTFV

SEQ ID NO: 4625 - protein, 9 aa, synthetic construct
GGDGNDSVD

SEQ ID NO: 4626 - protein, 9 aa, synthetic construct
GGDGDDEII

SEQ ID NO: 4627 - protein, 9 aa, synthetic construct
GGAGSDKLY

SEQ ID NO: 4628 - protein, 9 aa, synthetic construct
GGSGNDRMD

SEQ ID NO: 4629 - protein, 9 aa, synthetic construct
GGAGDDLME

SEQ ID NO: 4630 - protein, 9 aa, synthetic construct
GGLGDDTYL

SEQ ID NO: 4631 - protein, 9 aa, synthetic construct
GGAGSDMLI

SEQ ID NO: 4632 - protein, 9 aa, synthetic construct
GGRGSDTYR

SEQ ID NO: 4633 - protein, 9 aa, synthetic construct
GGAGNDQIY

SEQ ID NO: 4634 - protein, 9 aa, synthetic construct
GGAGDDQIR

SEQ ID NO: 4635 - protein, 9 aa, synthetic construct
GGLGDDILH

SEQ ID NO: 4636 - protein, 9 aa, synthetic construct
GGIGDDVLD

SEQ ID NO: 4637 - protein, 9 aa, synthetic construct
GGEGEDTLS

SEQ ID NO: 4638 - protein, 9 aa, synthetic construct
GGAGDDMLF

SEQ ID NO: 4639 - protein, 9 aa, synthetic construct
GGEGHDTLL

SEQ ID NO: 4640 - protein, 9 aa, synthetic construct
GGDGDDVIT

SEQ ID NO: 4641 - protein, 9 aa, synthetic construct
GGVGADSLI

SEQ ID NO: 4642 - protein, 9 aa, synthetic construct
GGDGDDRMW

SEQ ID NO: 4643 - protein, 9 aa, synthetic construct
GGYGDDILD

SEQ ID NO: 4644 - protein, 9 aa, synthetic construct
GGAGDDTFL

SEQ ID NO: 4645 - protein, 9 aa, synthetic construct
GGEGNDYIH

SEQ ID NO: 4646 - protein, 9 aa, synthetic construct
GGTGEDIFK

SEQ ID NO: 4647 - protein, 9 aa, synthetic construct
GGDGNDLIE

SEQ ID NO: 4648 - protein, 9 aa, synthetic construct
GGDGDDIVR

SEQ ID NO: 4649 - protein, 9 aa, synthetic construct
GGNGNDFIS

SEQ ID NO: 4650 - protein, 9 aa, synthetic construct
GGSGDDLLA

SEQ ID NO: 4651 - protein, 9 aa, synthetic construct
GGGGADSMT

SEQ ID NO: 4652 - protein, 9 aa, synthetic construct
GGEGNDILA

SEQ ID NO: 4653 - protein, 9 aa, synthetic construct
GGAGSDVLK

SEQ ID NO: 4654 - protein, 9 aa, synthetic construct
GGAGRDKLY

SEQ ID NO: 4655 - protein, 9 aa, synthetic construct
GGIGNDRLE

SEQ ID NO: 4656 - protein, 9 aa, synthetic construct
GGGGDDTLQ

SEQ ID NO: 4657 - protein, 9 aa, synthetic construct
GGTGNDFLV

SEQ ID NO: 4658 - protein, 9 aa, synthetic construct
GGSGHDTLQ

SEQ ID NO: 4659 - protein, 9 aa, synthetic construct
GGGGNDVIL

SEQ ID NO: 4660 - protein, 9 aa, synthetic construct
GGAGQDTFV

SEQ ID NO: 4661 - protein, 9 aa, synthetic construct
GGSGNDLVR

SEQ ID NO: 4662 - protein, 9 aa, synthetic construct
GGAGNDALE

SEQ ID NO: 4663 - protein, 9 aa, synthetic construct
GGAGDDHLI

SEQ ID NO: 4664 - protein, 9 aa, synthetic construct
GGQGSDTLD

SEQ ID NO: 4665 - protein, 9 aa, synthetic construct
GGAGNDILG

SEQ ID NO: 4666 - protein, 9 aa, synthetic construct
GGTGNDYLA

SEQ ID NO: 4667 - protein, 9 aa, synthetic construct
GGNGHDTLI

SEQ ID NO: 4668 - protein, 9 aa, synthetic construct
GGAGDDRIQ

SEQ ID NO: 4669 - protein, 9 aa, synthetic construct
GGSGRDLLI

SEQ ID NO: 4670 - protein, 9 aa, synthetic construct
GGTGNDYLI

SEQ ID NO: 4671 - protein, 9 aa, synthetic construct
GGEGNDTIA

SEQ ID NO: 4672 - protein, 9 aa, synthetic construct
GGPGGDAFV

SEQ ID NO: 4673 - protein, 9 aa, synthetic construct
GGDGTDTLI

SEQ ID NO: 4674 - protein, 9 aa, synthetic construct
GGGGADLIF

SEQ ID NO: 4675 - protein, 9 aa, synthetic construct
GGTGDDQLY

SEQ ID NO: 4676 - protein, 9 aa, synthetic construct
GGDGSDRLY

SEQ ID NO: 4677 - protein, 9 aa, synthetic construct
GGTGNDFLA

SEQ ID NO: 4678 - protein, 9 aa, synthetic construct
GGAGNDRVD

SEQ ID NO: 4679 - protein, 9 aa, synthetic construct
GGAGRDLIG

SEQ ID NO: 4680 - protein, 9 aa, synthetic construct
GGAGDDGLY

SEQ ID NO: 4681 - protein, 9 aa, synthetic construct
GGNGADRLL

SEQ ID NO: 4682 - protein, 9 aa, synthetic construct
GGGGSDILI

SEQ ID NO: 4683 - protein, 9 aa, synthetic construct
GGLGKDSLT

SEQ ID NO: 4684 - protein, 9 aa, synthetic construct
GGDGSDSVE

SEQ ID NO: 4685 - protein, 9 aa, synthetic construct
GGLGADVLL

SEQ ID NO: 4686 - protein, 9 aa, synthetic construct
GGVGIDSME

SEQ ID NO: 4687 - protein, 9 aa, synthetic construct
GGLGNDDLA

SEQ ID NO: 4688 - protein, 9 aa, synthetic construct
GGRGNDRLT

SEQ ID NO: 4689 - protein, 9 aa, synthetic construct
GGIGDDTLE

SEQ ID NO: 4690 - protein, 9 aa, synthetic construct
GGAGNDSYI

SEQ ID NO: 4691 - protein, 9 aa, synthetic construct
GGDGNDYLE

SEQ ID NO: 4692 - protein, 9 aa, synthetic construct
GGSGRDTLL

SEQ ID NO: 4693 - protein, 9 aa, synthetic construct
GGQGRDRME

SEQ ID NO: 4694 - protein, 9 aa, synthetic construct
GGAGMDTLS

SEQ ID NO: 4695 - protein, 9 aa, synthetic construct
GGTGRDTLS

SEQ ID NO: 4696 - protein, 9 aa, synthetic construct
GGDGDDALQ

SEQ ID NO: 4697 - protein, 9 aa, synthetic construct
GGEGDDVFD

SEQ ID NO: 4698 - protein, 9 aa, synthetic construct
GGSGRDTLA

SEQ ID NO: 4699 - protein, 9 aa, synthetic construct
GGAGKDTMT

SEQ ID NO: 4700 - protein, 9 aa, synthetic construct
GGNGSDFIV

SEQ ID NO: 4701 - protein, 9 aa, synthetic construct
GGTGNDVYV

SEQ ID NO: 4702 - protein, 9 aa, synthetic construct
GGNGNDVFV

SEQ ID NO: 4703 - protein, 9 aa, synthetic construct
GGGGNDKLN

SEQ ID NO: 4704 - protein, 9 aa, synthetic construct
GGDGDDMLV

SEQ ID NO: 4705 - protein, 9 aa, synthetic construct
GGNGHDIIY

SEQ ID NO: 4706 - protein, 9 aa, synthetic construct
GGAGNDFLV

SEQ ID NO: 4707 - protein, 9 aa, synthetic construct
GGTGVDTLY

SEQ ID NO: 4708 - protein, 9 aa, synthetic construct
GGQGSDTLT

SEQ ID NO: 4709 - protein, 9 aa, synthetic construct
GGAGQDSLY

SEQ ID NO: 4710 - protein, 9 aa, synthetic construct
GGQGDDTLV

SEQ ID NO: 4711 - protein, 9 aa, synthetic construct
GGLGNDVYI

SEQ ID NO: 4712 - protein, 9 aa, synthetic construct
GGDGTDTLY

SEQ ID NO: 4713 - protein, 9 aa, synthetic construct
GGQGDDVLV

SEQ ID NO: 4714 - protein, 9 aa, synthetic construct
GGAGNDAIF

SEQ ID NO: 4715 - protein, 9 aa, synthetic construct
GGDGDDSIY

SEQ ID NO: 4716 - protein, 9 aa, synthetic construct
GGSGSDILR

SEQ ID NO: 4717 - protein, 9 aa, synthetic construct
GGGGDDFLF

SEQ ID NO: 4718 - protein, 9 aa, synthetic construct
GGAGNDVVR

SEQ ID NO: 4719 - protein, 9 aa, synthetic construct
GGAGADSLH

SEQ ID NO: 4720 - protein, 9 aa, synthetic construct
GGAGKDMLS

SEQ ID NO: 4721 - protein, 9 aa, synthetic construct
GGNGRDTLL

SEQ ID NO: 4722 - protein, 9 aa, synthetic construct
GGEGNDKLF

SEQ ID NO: 4723 - protein, 9 aa, synthetic construct
GGDGADSIS

SEQ ID NO: 4724 - protein, 9 aa, synthetic construct
GGNGRDTLA

SEQ ID NO: 4725 - protein, 9 aa, synthetic construct
GGDGDDFIY

SEQ ID NO: 4726 - protein, 9 aa, synthetic construct
GGEGDDLLF

SEQ ID NO: 4727 - protein, 9 aa, synthetic construct
GGTGADTMN

SEQ ID NO: 4728 - protein, 9 aa, synthetic construct
GGGGSDMLS

SEQ ID NO: 4729 - protein, 9 aa, synthetic construct
GGLGADSLS

SEQ ID NO: 4730 - protein, 9 aa, synthetic construct
GGGGADIIL

SEQ ID NO: 4731 - protein, 9 aa, synthetic construct
GGYGNDILS

SEQ ID NO: 4732 - protein, 9 aa, synthetic construct
GGYGNDILV

SEQ ID NO: 4733 - protein, 9 aa, synthetic construct
GGAGQDYLN

SEQ ID NO: 4734 - protein, 9 aa, synthetic construct
GGQGADTLL

SEQ ID NO: 4735 - protein, 9 aa, synthetic construct
GGQGADTLF

SEQ ID NO: 4736 - protein, 9 aa, synthetic construct
GGAGTDILI

SEQ ID NO: 4737 - protein, 9 aa, synthetic construct
GGEGNDVIF

SEQ ID NO: 4738 - protein, 9 aa, synthetic construct
GGIGNDTID

SEQ ID NO: 4739 - protein, 9 aa, synthetic construct
GGSGSDTIR

SEQ ID NO: 4740 - protein, 9 aa, synthetic construct
GGEGNDVIL

SEQ ID NO: 4741 - protein, 9 aa, synthetic construct
GGAGADWLD

SEQ ID NO: 4742 - protein, 9 aa, synthetic construct
GGEGFDTAT

SEQ ID NO: 4743 - protein, 9 aa, synthetic construct
GGTGQDTLF

SEQ ID NO: 4744 - protein, 9 aa, synthetic construct
GGDGNDTAD

SEQ ID NO: 4745 - protein, 9 aa, synthetic construct
GGDGDDTFI

SEQ ID NO: 4746 - protein, 9 aa, synthetic construct
GGAGDDGLA

SEQ ID NO: 4747 - protein, 9 aa, synthetic construct
GGAGKDTLR

SEQ ID NO: 4748 - protein, 9 aa, synthetic construct
GGGGADSLS

SEQ ID NO: 4749 - protein, 9 aa, synthetic construct
GGDGIDNLQ

SEQ ID NO: 4750 - protein, 9 aa, synthetic construct
GGTGADVFA

SEQ ID NO: 4751 - protein, 9 aa, synthetic construct
GGNGADRLY

SEQ ID NO: 4752 - protein, 9 aa, synthetic construct
GGEGADTMI

SEQ ID NO: 4753 - protein, 9 aa, synthetic construct
GGAGHDVLW

SEQ ID NO: 4754 - protein, 9 aa, synthetic construct
GGAGQDTLN

SEQ ID NO: 4755 - protein, 9 aa, synthetic construct
GGLGADTME

SEQ ID NO: 4756 - protein, 9 aa, synthetic construct
GGAGNDHLE

SEQ ID NO: 4757 - protein, 9 aa, synthetic construct
GGGGSDTIY

SEQ ID NO: 4758 - protein, 9 aa, synthetic construct
GGGGGDTLN

SEQ ID NO: 4759 - protein, 9 aa, synthetic construct
GGPGADTLI

SEQ ID NO: 4760 - protein, 9 aa, synthetic construct
GGDGCDVLI

SEQ ID NO: 4761 - protein, 9 aa, synthetic construct
GGLGVDTLI

SEQ ID NO: 4762 - protein, 9 aa, synthetic construct
GGKGKDVFV

SEQ ID NO: 4763 - protein, 9 aa, synthetic construct
GGGGSDNMR

SEQ ID NO: 4764 - protein, 9 aa, synthetic construct
GGAGNDVMN

SEQ ID NO: 4765 - protein, 9 aa, synthetic construct
GGNGHDLLR

SEQ ID NO: 4766 - protein, 9 aa, synthetic construct
GGAGDDFLH

SEQ ID NO: 4767 - protein, 9 aa, synthetic construct
GGFGADSLS

SEQ ID NO: 4768 - protein, 9 aa, synthetic construct
GGDGNDRLW

SEQ ID NO: 4769 - protein, 9 aa, synthetic construct
GGAGFDRLF

SEQ ID NO: 4770 - protein, 9 aa, synthetic construct
GGPGADVIH

SEQ ID NO: 4771 - protein, 9 aa, synthetic construct
GGSGDDSLN

SEQ ID NO: 4772 - protein, 9 aa, synthetic construct
GGAGTDLIL

SEQ ID NO: 4773 - protein, 9 aa, synthetic construct
GGDGDDNLD

SEQ ID NO: 4774 - protein, 9 aa, synthetic construct
GGAGADSLQ

SEQ ID NO: 4775 - protein, 9 aa, synthetic construct
GGDGNDEIS

SEQ ID NO: 4776 - protein, 9 aa, synthetic construct
GGGGADKLS

SEQ ID NO: 4777 - protein, 9 aa, synthetic construct
GGGGDDRLV

SEQ ID NO: 4778 - protein, 9 aa, synthetic construct
GGDGNDMLS

SEQ ID NO: 4779 - protein, 9 aa, synthetic construct
GGEGDDRLV

SEQ ID NO: 4780 - protein, 9 aa, synthetic construct
GGAGGDRLL

SEQ ID NO: 4781 - protein, 9 aa, synthetic construct
GGRGDDRLE

SEQ ID NO: 4782 - protein, 9 aa, synthetic construct
GGSGDDTFA

SEQ ID NO: 4783 - protein, 9 aa, synthetic construct
GGPGDDSIG

SEQ ID NO: 4784 - protein, 9 aa, synthetic construct
GGEGNDIII

SEQ ID NO: 4785 - protein, 9 aa, synthetic construct
GGAGNDELF

SEQ ID NO: 4786 - protein, 9 aa, synthetic construct
GGGGDDSID

SEQ ID NO: 4787 - protein, 9 aa, synthetic construct
GGDGVDVLI

SEQ ID NO: 4788 - protein, 9 aa, synthetic construct
GGSGSDYLN

SEQ ID NO: 4789 - protein, 9 aa, synthetic construct
GGSGNDSLE

SEQ ID NO: 4790 - protein, 9 aa, synthetic construct
GGAGSDTIS

SEQ ID NO: 4791 - protein, 9 aa, synthetic construct
GGTGNDTMD

SEQ ID NO: 4792 - protein, 9 aa, synthetic construct
GGTGDDTVD

SEQ ID NO: 4793 - protein, 9 aa, synthetic construct
GGSGRDRLE

SEQ ID NO: 4794 - protein, 9 aa, synthetic construct
GGRGNDTLF

SEQ ID NO: 4795 - protein, 9 aa, synthetic construct
GGSGNDAVA

SEQ ID NO: 4796 - protein, 9 aa, synthetic construct
GGDGDDWLY

SEQ ID NO: 4797 - protein, 9 aa, synthetic construct
GGTGNDTML

SEQ ID NO: 4798 - protein, 9 aa, synthetic construct
GGVGFDTLT

SEQ ID NO: 4799 - protein, 9 aa, synthetic construct
GGTGNDTMS

SEQ ID NO: 4800 - protein, 9 aa, synthetic construct
GGSGNDTMS

SEQ ID NO: 4801 - protein, 9 aa, synthetic construct
GGRGNDTLA

SEQ ID NO: 4802 - protein, 9 aa, synthetic construct
GGIGNDLLQ

SEQ ID NO: 4803 - protein, 9 aa, synthetic construct
GGAGDDWLY

SEQ ID NO: 4804 - protein, 9 aa, synthetic construct
GGDGDDVMT

SEQ ID NO: 4805 - protein, 9 aa, synthetic construct
GGAGSDTLQ

SEQ ID NO: 4806 - protein, 9 aa, synthetic construct
GGTGNDTLG

SEQ ID NO: 4807 - protein, 9 aa, synthetic construct
GGAGSDTIF

SEQ ID NO: 4808 - protein, 9 aa, synthetic construct
GGVGADLLG

SEQ ID NO: 4809 - protein, 9 aa, synthetic construct
GGAGVDKLV

SEQ ID NO: 4810 - protein, 9 aa, synthetic construct
GGAGADIVF

SEQ ID NO: 4811 - protein, 9 aa, synthetic construct
GGSGDDALY

SEQ ID NO: 4812 - protein, 9 aa, synthetic construct
GGGGRDLLI

SEQ ID NO: 4813 - protein, 9 aa, synthetic construct
GGAGNDSVY

SEQ ID NO: 4814 - protein, 9 aa, synthetic construct
GGTGADYLN

SEQ ID NO: 4815 - protein, 9 aa, synthetic construct
GGAGNDLLG

SEQ ID NO: 4816 - protein, 9 aa, synthetic construct
GGAGNDQMG

SEQ ID NO: 4817 - protein, 9 aa, synthetic construct
GGAGSDSLL

SEQ ID NO: 4818 - protein, 9 aa, synthetic construct
GGAGADTIL

SEQ ID NO: 4819 - protein, 9 aa, synthetic construct
GGAGADYLS

SEQ ID NO: 4820 - protein, 9 aa, synthetic construct
GGGGDDSLF

SEQ ID NO: 4821 - protein, 9 aa, synthetic construct
GGTGADLLN

SEQ ID NO: 4822 - protein, 9 aa, synthetic construct
GGSGNDIIV

SEQ ID NO: 4823 - protein, 9 aa, synthetic construct
GGRGNDTMS

SEQ ID NO: 4824 - protein, 9 aa, synthetic construct
GGRGNDTLV

SEQ ID NO: 4825 - protein, 9 aa, synthetic construct
GGDGNDNLY

SEQ ID NO: 4826 - protein, 9 aa, synthetic construct
GGSGQDTMT

SEQ ID NO: 4827 - protein, 9 aa, synthetic construct
GGDGNDQLS

SEQ ID NO: 4828 - protein, 9 aa, synthetic construct
GGAGFDTLF

SEQ ID NO: 4829 - protein, 9 aa, synthetic construct
GGAGADIMH

SEQ ID NO: 4830 - protein, 9 aa, synthetic construct
GGGGDDLLR

SEQ ID NO: 4831 - protein, 9 aa, synthetic construct
GGNGNDTVL

SEQ ID NO: 4832 - protein, 9 aa, synthetic construct
GGDGLDLAI

SEQ ID NO: 4833 - protein, 9 aa, synthetic construct
GGAGSDTFL

SEQ ID NO: 4834 - protein, 9 aa, synthetic construct
GGAGIDTFV

SEQ ID NO: 4835 - protein, 9 aa, synthetic construct
GGSGDDFLA

SEQ ID NO: 4836 - protein, 9 aa, synthetic construct
GGGGADRLT

SEQ ID NO: 4837 - protein, 9 aa, synthetic construct
GGGGNDFLS

SEQ ID NO: 4838 - protein, 9 aa, synthetic construct
GGLGADVMT

SEQ ID NO: 4839 - protein, 9 aa, synthetic construct
GGAGDDYLA

SEQ ID NO: 4840 - protein, 9 aa, synthetic construct
GGLGDDQIL

SEQ ID NO: 4841 - protein, 9 aa, synthetic construct
GGKGKDFFI

SEQ ID NO: 4842 - protein, 9 aa, synthetic construct
GGSGDDILA

SEQ ID NO: 4843 - protein, 9 aa, synthetic construct
GGLGEDMLN

SEQ ID NO: 4844 - protein, 9 aa, synthetic construct
GGTGDDRLE

SEQ ID NO: 4845 - protein, 9 aa, synthetic construct
GGAGADTFQ

SEQ ID NO: 4846 - protein, 9 aa, synthetic construct
GGAGSDFYV

SEQ ID NO: 4847 - protein, 9 aa, synthetic construct
GGAGGDSLY

SEQ ID NO: 4848 - protein, 9 aa, synthetic construct
GGAGDDSIR

SEQ ID NO: 4849 - protein, 9 aa, synthetic construct
GGKGNDKLN

SEQ ID NO: 4850 - protein, 9 aa, synthetic construct
GGGGNDILS

SEQ ID NO: 4851 - protein, 9 aa, synthetic construct
GGVGNDTLK

SEQ ID NO: 4852 - protein, 9 aa, synthetic construct
GGAGADMLA

SEQ ID NO: 4853 - protein, 9 aa, synthetic construct
GGSGNDTML

SEQ ID NO: 4854 - protein, 9 aa, synthetic construct
GGTGNDGLY

SEQ ID NO: 4855 - protein, 9 aa, synthetic construct
GGEGDDSLA

SEQ ID NO: 4856 - protein, 9 aa, synthetic construct
GGSGSDSLD

SEQ ID NO: 4857 - protein, 9 aa, synthetic construct
GGGGLDTLI

SEQ ID NO: 4858 - protein, 9 aa, synthetic construct
GGAGTDRFL

SEQ ID NO: 4859 - protein, 9 aa, synthetic construct
GGAGDDSIL

SEQ ID NO: 4860 - protein, 9 aa, synthetic construct
GGLGNDTFF

SEQ ID NO: 4861 - protein, 9 aa, synthetic construct
GGPGDDTLL

SEQ ID NO: 4862 - protein, 9 aa, synthetic construct
GGEGDDRLL

SEQ ID NO: 4863 - protein, 9 aa, synthetic construct
GGSGSDQIV

SEQ ID NO: 4864 - protein, 9 aa, synthetic construct
GGDGADVLL

SEQ ID NO: 4865 - protein, 9 aa, synthetic construct
GGTGNDVLQ

SEQ ID NO: 4866 - protein, 9 aa, synthetic construct
GGTGNDTVS

SEQ ID NO: 4867 - protein, 9 aa, synthetic construct
GGRGNDTIF

SEQ ID NO: 4868 - protein, 9 aa, synthetic construct
GGGGADRLV

SEQ ID NO: 4869 - protein, 9 aa, synthetic construct
GGGGNDFLY

SEQ ID NO: 4870 - protein, 9 aa, synthetic construct
GGVGADKLL

SEQ ID NO: 4871 - protein, 9 aa, synthetic construct
GGDGDDRLM

SEQ ID NO: 4872 - protein, 9 aa, synthetic construct
GGEGNDLIA

SEQ ID NO: 4873 - protein, 9 aa, synthetic construct
GGAGDDYLH

SEQ ID NO: 4874 - protein, 9 aa, synthetic construct
GGAGDDDLW

SEQ ID NO: 4875 - protein, 9 aa, synthetic construct
GGTGDDLYA

SEQ ID NO: 4876 - protein, 9 aa, synthetic construct
GGAGFDTLT

SEQ ID NO: 4877 - protein, 9 aa, synthetic construct
GGTGADILI

SEQ ID NO: 4878 - protein, 9 aa, synthetic construct
GGAGADYMA

SEQ ID NO: 4879 - protein, 9 aa, synthetic construct
GGAGDDQLN

SEQ ID NO: 4880 - protein, 9 aa, synthetic construct
GGEGDDDLF

SEQ ID NO: 4881 - protein, 9 aa, synthetic construct
GGGGADSLF

SEQ ID NO: 4882 - protein, 9 aa, synthetic construct
GGSGNDNLS

SEQ ID NO: 4883 - protein, 9 aa, synthetic construct
GGAGMDILT

SEQ ID NO: 4884 - protein, 9 aa, synthetic construct
GGNGNDILA

SEQ ID NO: 4885 - protein, 9 aa, synthetic construct
GGSGNDNII

SEQ ID NO: 4886 - protein, 9 aa, synthetic construct
GGHGSDSLD

SEQ ID NO: 4887 - protein, 9 aa, synthetic construct
GGTGLDTLI

SEQ ID NO: 4888 - protein, 9 aa, synthetic construct
GGSGADFIN

SEQ ID NO: 4889 - protein, 9 aa, synthetic construct
GGGGADTIN

SEQ ID NO: 4890 - protein, 9 aa, synthetic construct
GGTGQDTIR

SEQ ID NO: 4891 - protein, 9 aa, synthetic construct
GGTGADIFR

SEQ ID NO: 4892 - protein, 9 aa, synthetic construct
GGAGFDTLV

SEQ ID NO: 4893 - protein, 9 aa, synthetic construct
GGKGSDFLD

SEQ ID NO: 4894 - protein, 9 aa, synthetic construct
GGDGDDSLE

SEQ ID NO: 4895 - protein, 9 aa, synthetic construct
GGNGADSLL

SEQ ID NO: 4896 - protein, 9 aa, synthetic construct
GGAGFDTLN

SEQ ID NO: 4897 - protein, 9 aa, synthetic construct
GGAGADYLA

SEQ ID NO: 4898 - protein, 9 aa, synthetic construct
GGGGADTFA

SEQ ID NO: 4899 - protein, 9 aa, synthetic construct
GGMGDDSLD

SEQ ID NO: 4900 - protein, 9 aa, synthetic construct
GGPGNDVFV

SEQ ID NO: 4901 - protein, 9 aa, synthetic construct
GGAGNDKLR

SEQ ID NO: 4902 - protein, 9 aa, synthetic construct
GGDGNDLFI

SEQ ID NO: 4903 - protein, 9 aa, synthetic construct
GGSGTDTLN

SEQ ID NO: 4904 - protein, 9 aa, synthetic construct
GGSGTDTAD

SEQ ID NO: 4905 - protein, 9 aa, synthetic construct
GGGGDDLID

SEQ ID NO: 4906 - protein, 9 aa, synthetic construct
GGLGSDTLR

SEQ ID NO: 4907 - protein, 9 aa, synthetic construct
GGDGNDQLV

SEQ ID NO: 4908 - protein, 9 aa, synthetic construct
GGEGADTFL

SEQ ID NO: 4909 - protein, 9 aa, synthetic construct
GGDGNDRLK

SEQ ID NO: 4910 - protein, 9 aa, synthetic construct
GGLGNDNLS

SEQ ID NO: 4911 - protein, 9 aa, synthetic construct
GGDGDDVIA

SEQ ID NO: 4912 - protein, 9 aa, synthetic construct
GGEGKDTLS

SEQ ID NO: 4913 - protein, 9 aa, synthetic construct
GGQGNDTLV

SEQ ID NO: 4914 - protein, 9 aa, synthetic construct
GGDGDDSIT

SEQ ID NO: 4915 - protein, 9 aa, synthetic construct
GGGGTDTLI

SEQ ID NO: 4916 - protein, 9 aa, synthetic construct
GGQGNDTLE

SEQ ID NO: 4917 - protein, 9 aa, synthetic construct
GGVGADSLF

SEQ ID NO: 4918 - protein, 9 aa, synthetic construct
GGQGRDILT

SEQ ID NO: 4919 - protein, 9 aa, synthetic construct
GGHGSDTIY

SEQ ID NO: 4920 - protein, 9 aa, synthetic construct
GGAGNDQLW

SEQ ID NO: 4921 - protein, 9 aa, synthetic construct
GGGGSDRLV

SEQ ID NO: 4922 - protein, 9 aa, synthetic construct
GGAGNDVFL

SEQ ID NO: 4923 - protein, 9 aa, synthetic construct
GGNGNDILV

SEQ ID NO: 4924 - protein, 9 aa, synthetic construct
GGAGNDVMS

SEQ ID NO: 4925 - protein, 9 aa, synthetic construct
GGDGSDEIY

SEQ ID NO: 4926 - protein, 9 aa, synthetic construct
GGTGADHMA

SEQ ID NO: 4927 - protein, 9 aa, synthetic construct
GGLGNDLYQ

SEQ ID NO: 4928 - protein, 9 aa, synthetic construct
GGLGNDMFR

SEQ ID NO: 4929 - protein, 9 aa, synthetic construct
GGLGDDRLI

SEQ ID NO: 4930 - protein, 9 aa, synthetic construct
GGDGNDVIW

SEQ ID NO: 4931 - protein, 9 aa, synthetic construct
GGAGSDILR

SEQ ID NO: 4932 - protein, 9 aa, synthetic construct
GGAGNDLIA

SEQ ID NO: 4933 - protein, 9 aa, synthetic construct
GGLGNDQLD

SEQ ID NO: 4934 - protein, 9 aa, synthetic construct
GGDGNDLVD

SEQ ID NO: 4935 - protein, 9 aa, synthetic construct
GGSGNDQLL

SEQ ID NO: 4936 - protein, 9 aa, synthetic construct
GGAGDDIFR

SEQ ID NO: 4937 - protein, 9 aa, synthetic construct
GGSGRDTLS

SEQ ID NO: 4938 - protein, 9 aa, synthetic construct
GGLGSDFLI

SEQ ID NO: 4939 - protein, 9 aa, synthetic construct
GGSGKDIFV

SEQ ID NO: 4940 - protein, 9 aa, synthetic construct
GGAGNDIFK

SEQ ID NO: 4941 - protein, 9 aa, synthetic construct
GGEGSDLLD

SEQ ID NO: 4942 - protein, 9 aa, synthetic construct
GGNGSDLLL

SEQ ID NO: 4943 - protein, 9 aa, synthetic construct
GGVGNDTII

SEQ ID NO: 4944 - protein, 9 aa, synthetic construct
GGAGDDIIS

SEQ ID NO: 4945 - protein, 9 aa, synthetic construct
GGSGRDTLN

SEQ ID NO: 4946 - protein, 9 aa, synthetic construct
GGKGDDQLA

SEQ ID NO: 4947 - protein, 9 aa, synthetic construct
GGAGGDTLA

SEQ ID NO: 4948 - protein, 9 aa, synthetic construct
GGAGNDSIF

SEQ ID NO: 4949 - protein, 9 aa, synthetic construct
GGSGDDIMT

SEQ ID NO: 4950 - protein, 9 aa, synthetic construct
GGAGGDTLQ

SEQ ID NO: 4951 - protein, 9 aa, synthetic construct
GGSGRDTLF

SEQ ID NO: 4952 - protein, 9 aa, synthetic construct
GGAGNDRYE

SEQ ID NO: 4953 - protein, 9 aa, synthetic construct
GGAGSDVLA

SEQ ID NO: 4954 - protein, 9 aa, synthetic construct
GGDGTDTAS

SEQ ID NO: 4955 - protein, 9 aa, synthetic construct
GGQGDDTLY

SEQ ID NO: 4956 - protein, 9 aa, synthetic construct
GGTGADVLN

SEQ ID NO: 4957 - protein, 9 aa, synthetic construct
GGSGDDLLF

SEQ ID NO: 4958 - protein, 9 aa, synthetic construct
GGNGNDTIK

SEQ ID NO: 4959 - protein, 9 aa, synthetic construct
GGVGNDTLE

SEQ ID NO: 4960 - protein, 9 aa, synthetic construct
GGAGNDSIG

SEQ ID NO: 4961 - protein, 9 aa, synthetic construct
GGAGNDELL

SEQ ID NO: 4962 - protein, 9 aa, synthetic construct
GGTGGDYID

SEQ ID NO: 4963 - protein, 9 aa, synthetic construct
GGAGTDSLI

SEQ ID NO: 4964 - protein, 9 aa, synthetic construct
GGSGHDHLR

SEQ ID NO: 4965 - protein, 9 aa, synthetic construct
GGDGTDRIQ

SEQ ID NO: 4966 - protein, 9 aa, synthetic construct
GGSGDDFID

SEQ ID NO: 4967 - protein, 9 aa, synthetic construct
GGEGADNLL

SEQ ID NO: 4968 - protein, 9 aa, synthetic construct
GGAGSDTLE

SEQ ID NO: 4969 - protein, 9 aa, synthetic construct
GGSGDDFIV

SEQ ID NO: 4970 - protein, 9 aa, synthetic construct
GGVGNDTYT

SEQ ID NO: 4971 - protein, 9 aa, synthetic construct
GGVGNDTYH

SEQ ID NO: 4972 - protein, 9 aa, synthetic construct
GGAGDDDLS

SEQ ID NO: 4973 - protein, 9 aa, synthetic construct
GGDGDDLVS

SEQ ID NO: 4974 - protein, 9 aa, synthetic construct
GGDGGDTLS

SEQ ID NO: 4975 - protein, 9 aa, synthetic construct
GGAGADILE

SEQ ID NO: 4976 - protein, 9 aa, synthetic construct
GGAGKDILY

SEQ ID NO: 4977 - protein, 9 aa, synthetic construct
GGDGVDFLE

SEQ ID NO: 4978 - protein, 9 aa, synthetic construct
GGNGADVLD

SEQ ID NO: 4979 - protein, 9 aa, synthetic construct
GGAGHDIII

SEQ ID NO: 4980 - protein, 9 aa, synthetic construct
GGDGGDTLN

SEQ ID NO: 4981 - protein, 9 aa, synthetic construct
GGAGSDTVQ

SEQ ID NO: 4982 - protein, 9 aa, synthetic construct
GGAGADALR

SEQ ID NO: 4983 - protein, 9 aa, synthetic construct
GGLGEDILI

SEQ ID NO: 4984 - protein, 9 aa, synthetic construct
GGSGSDVYR

SEQ ID NO: 4985 - protein, 9 aa, synthetic construct
GGEGNDVLE

SEQ ID NO: 4986 - protein, 9 aa, synthetic construct
GGLGNDTIL

SEQ ID NO: 4987 - protein, 9 aa, synthetic construct
GGAGADHMR

SEQ ID NO: 4988 - protein, 9 aa, synthetic construct
GGEGRDFIF

SEQ ID NO: 4989 - protein, 9 aa, synthetic construct
GGSGDDSLV

SEQ ID NO: 4990 - protein, 9 aa, synthetic construct
GGGGRDRLF

SEQ ID NO: 4991 - protein, 9 aa, synthetic construct
GGDGDDWIE

SEQ ID NO: 4992 - protein, 9 aa, synthetic construct
GGVGNDIYH

SEQ ID NO: 4993 - protein, 9 aa, synthetic construct
GGEGDDVLE

SEQ ID NO: 4994 - protein, 9 aa, synthetic construct
GGAGDDELD

SEQ ID NO: 4995 - protein, 9 aa, synthetic construct
GGDGNDVVS

SEQ ID NO: 4996 - protein, 9 aa, synthetic construct
GGAGDDFIS

SEQ ID NO: 4997 - protein, 9 aa, synthetic construct
GGAGDDFIQ

SEQ ID NO: 4998 - protein, 9 aa, synthetic construct
GGAGDDELF

SEQ ID NO: 4999 - protein, 9 aa, synthetic construct
GGEGDDFID

SEQ ID NO: 5000 - protein, 9 aa, synthetic construct
GGGGLDVID

SEQ ID NO: 5001 - protein, 9 aa, synthetic construct
GGDGDDRIE

SEQ ID NO: 5002 - protein, 9 aa, synthetic construct
GGVGNDLLQ

SEQ ID NO: 5003 - protein, 9 aa, synthetic construct
GGAGTDILD

SEQ ID NO: 5004 - protein, 9 aa, synthetic construct
GGAGNDRFD

SEQ ID NO: 5005 - protein, 9 aa, synthetic construct
GGGGRDRLT

SEQ ID NO: 5006 - protein, 9 aa, synthetic construct
GGLGNDTMV

SEQ ID NO: 5007 - protein, 9 aa, synthetic construct
GGQGADTFV

SEQ ID NO: 5008 - protein, 9 aa, synthetic construct
GGLGGDTMT

SEQ ID NO: 5009 - protein, 9 aa, synthetic construct
GGKGNDTYY

SEQ ID NO: 5010 - protein, 9 aa, synthetic construct
GGEGDDFLF

SEQ ID NO: 5011 - protein, 9 aa, synthetic construct
GGVGNDRLI

SEQ ID NO: 5012 - protein, 9 aa, synthetic construct
GGAGDDFLT

SEQ ID NO: 5013 - protein, 9 aa, synthetic construct
GGAGADAID

SEQ ID NO: 5014 - protein, 9 aa, synthetic construct
GGIGNDSLN

SEQ ID NO: 5015 - protein, 9 aa, synthetic construct
GGAGDDHLE

SEQ ID NO: 5016 - protein, 9 aa, synthetic construct
GGQGDDSLS

SEQ ID NO: 5017 - protein, 9 aa, synthetic construct
GGEGNDALY

SEQ ID NO: 5018 - protein, 9 aa, synthetic construct
GGQGDDSLI

SEQ ID NO: 5019 - protein, 9 aa, synthetic construct
GGDGNDTYF

SEQ ID NO: 5020 - protein, 9 aa, synthetic construct
GGDGTDTLD

SEQ ID NO: 5021 - protein, 9 aa, synthetic construct
GGNGNDTIA

SEQ ID NO: 5022 - protein, 9 aa, synthetic construct
GGAGNDRMI

SEQ ID NO: 5023 - protein, 9 aa, synthetic construct
GGEGIDRAV

SEQ ID NO: 5024 - protein, 9 aa, synthetic construct
GGDGDDRIY

SEQ ID NO: 5025 - protein, 9 aa, synthetic construct
GGDGDDVVR

SEQ ID NO: 5026 - protein, 9 aa, synthetic construct
GGAGSDYAL

SEQ ID NO: 5027 - protein, 9 aa, synthetic construct
GGGGNDALN

SEQ ID NO: 5028 - protein, 9 aa, synthetic construct
GGGGNDRIR

SEQ ID NO: 5029 - protein, 9 aa, synthetic construct
GGGGDDALD

SEQ ID NO: 5030 - protein, 9 aa, synthetic construct
GGAGNDFVN

SEQ ID NO: 5031 - protein, 9 aa, synthetic construct
GGDGADQLD

SEQ ID NO: 5032 - protein, 9 aa, synthetic construct
GGSGNDTIA

SEQ ID NO: 5033 - protein, 9 aa, synthetic construct
GGVGNDFLY

SEQ ID NO: 5034 - protein, 9 aa, synthetic construct
GGEGDDTLM

SEQ ID NO: 5035 - protein, 9 aa, synthetic construct
GGAGDDFVA

SEQ ID NO: 5036 - protein, 9 aa, synthetic construct
GGDGADLLC

SEQ ID NO: 5037 - protein, 9 aa, synthetic construct
GGEGDDRMW

SEQ ID NO: 5038 - protein, 9 aa, synthetic construct
GGAGDDKLE

SEQ ID NO: 5039 - protein, 9 aa, synthetic construct
GGVGDDQLY

SEQ ID NO: 5040 - protein, 9 aa, synthetic construct
GGDGRDTLR

SEQ ID NO: 5041 - protein, 9 aa, synthetic construct
GGAGADLFL

SEQ ID NO: 5042 - protein, 9 aa, synthetic construct
GGLGNDRIF

SEQ ID NO: 5043 - protein, 9 aa, synthetic construct
GGNGADTLR

SEQ ID NO: 5044 - protein, 9 aa, synthetic construct
GGVGDDLLD

SEQ ID NO: 5045 - protein, 9 aa, synthetic construct
GGEGNDFLY

SEQ ID NO: 5046 - protein, 9 aa, synthetic construct
GGGGDDIID

SEQ ID NO: 5047 - protein, 9 aa, synthetic construct
GGVGDDQIF

SEQ ID NO: 5048 - protein, 9 aa, synthetic construct
GGLGVDTFK

SEQ ID NO: 5049 - protein, 9 aa, synthetic construct
GGLGRDILT

SEQ ID NO: 5050 - protein, 9 aa, synthetic construct
GGAGTDTVR

SEQ ID NO: 5051 - protein, 9 aa, synthetic construct
GGDGDDVLQ

SEQ ID NO: 5052 - protein, 9 aa, synthetic construct
GGQGNDELD

SEQ ID NO: 5053 - protein, 9 aa, synthetic construct
GGTGIDTAV

SEQ ID NO: 5054 - protein, 9 aa, synthetic construct
GGAGGDILS

SEQ ID NO: 5055 - protein, 9 aa, synthetic construct
GGSGSDRLE

SEQ ID NO: 5056 - protein, 9 aa, synthetic construct
GGGGDDIFV

SEQ ID NO: 5057 - protein, 9 aa, synthetic construct
GGGGRDTFT

SEQ ID NO: 5058 - protein, 9 aa, synthetic construct
GGKGNDIFV

SEQ ID NO: 5059 - protein, 9 aa, synthetic construct
GGYGDDTLS

SEQ ID NO: 5060 - protein, 9 aa, synthetic construct
GGGGGDTLV

SEQ ID NO: 5061 - protein, 9 aa, synthetic construct
GGSGADTYV

SEQ ID NO: 5062 - protein, 9 aa, synthetic construct
GGAGADAMT

SEQ ID NO: 5063 - protein, 9 aa, synthetic construct
GGEGNDTLM

SEQ ID NO: 5064 - protein, 9 aa, synthetic construct
GGYGDDLLD

SEQ ID NO: 5065 - protein, 9 aa, synthetic construct
GGVGDDIYL

SEQ ID NO: 5066 - protein, 9 aa, synthetic construct
GGLGDDSLF

SEQ ID NO: 5067 - protein, 9 aa, synthetic construct
GGIGRDRIN

SEQ ID NO: 5068 - protein, 9 aa, synthetic construct
GGMGKDVLT

SEQ ID NO: 5069 - protein, 9 aa, synthetic construct
GGLGDDSLL

SEQ ID NO: 5070 - protein, 9 aa, synthetic construct
GGAGGDAME

SEQ ID NO: 5071 - protein, 9 aa, synthetic construct
GGDGADTLG

SEQ ID NO: 5072 - protein, 9 aa, synthetic construct
GGDGGDLLD

SEQ ID NO: 5073 - protein, 9 aa, synthetic construct
GGSGADRMT

SEQ ID NO: 5074 - protein, 9 aa, synthetic construct
GGAGSDLLS

SEQ ID NO: 5075 - protein, 9 aa, synthetic construct
GGDGRDVIH

SEQ ID NO: 5076 - protein, 9 aa, synthetic construct
GGDGDDDIS

SEQ ID NO: 5077 - protein, 9 aa, synthetic construct
GGAGTDVLT

SEQ ID NO: 5078 - protein, 9 aa, synthetic construct
GGAGTDVLN

SEQ ID NO: 5079 - protein, 9 aa, synthetic construct
GGDGDDVIV

SEQ ID NO: 5080 - protein, 9 aa, synthetic construct
GGSGADSLT

SEQ ID NO: 5081 - protein, 9 aa, synthetic construct
GGVGDDILV

SEQ ID NO: 5082 - protein, 9 aa, synthetic construct
GGTGKDLLD

SEQ ID NO: 5083 - protein, 9 aa, synthetic construct
GGKGDDRLT

SEQ ID NO: 5084 - protein, 9 aa, synthetic construct
GGAGDDMIV

SEQ ID NO: 5085 - protein, 9 aa, synthetic construct
GGTGKDIMT

SEQ ID NO: 5086 - protein, 9 aa, synthetic construct
GGAGADLIF

SEQ ID NO: 5087 - protein, 9 aa, synthetic construct
GGQGLDSVF

SEQ ID NO: 5088 - protein, 9 aa, synthetic construct
GGDGADILV

SEQ ID NO: 5089 - protein, 9 aa, synthetic construct
GGLGSDTFT

SEQ ID NO: 5090 - protein, 9 aa, synthetic construct
GGNGSDTFV

SEQ ID NO: 5091 - protein, 9 aa, synthetic construct
GGTGHDSLL

SEQ ID NO: 5092 - protein, 9 aa, synthetic construct
GGAGNDSVS

SEQ ID NO: 5093 - protein, 9 aa, synthetic construct
GGFGSDTYV

SEQ ID NO: 5094 - protein, 9 aa, synthetic construct
GGAGSDSLV

SEQ ID NO: 5095 - protein, 9 aa, synthetic construct
GGMGNDVLH

SEQ ID NO: 5096 - protein, 9 aa, synthetic construct
GGGGADVLS

SEQ ID NO: 5097 - protein, 9 aa, synthetic construct
GGTGADLLR

SEQ ID NO: 5098 - protein, 9 aa, synthetic construct
GGAGADALV

SEQ ID NO: 5099 - protein, 9 aa, synthetic construct
GGKGDDYLE

SEQ ID NO: 5100 - protein, 9 aa, synthetic construct
GGAGNDFIH

SEQ ID NO: 5101 - protein, 9 aa, synthetic construct
GGLGNDSLV

SEQ ID NO: 5102 - protein, 9 aa, synthetic construct
GGVGDDTID

SEQ ID NO: 5103 - protein, 9 aa, synthetic construct
GGAGNDIMT

SEQ ID NO: 5104 - protein, 9 aa, synthetic construct
GGIGNDLFV

SEQ ID NO: 5105 - protein, 9 aa, synthetic construct
GGDGDDRLW

SEQ ID NO: 5106 - protein, 9 aa, synthetic construct
GGKGNDFLS

SEQ ID NO: 5107 - protein, 9 aa, synthetic construct
GGAGNDIMN

SEQ ID NO: 5108 - protein, 9 aa, synthetic construct
GGDGFDFLN

SEQ ID NO: 5109 - protein, 9 aa, synthetic construct
GGSGDDELD

SEQ ID NO: 5110 - protein, 9 aa, synthetic construct
GGSGNDTVI

SEQ ID NO: 5111 - protein, 9 aa, synthetic construct
GGAGDDKLS

SEQ ID NO: 5112 - protein, 9 aa, synthetic construct
GGAGGDRLH

SEQ ID NO: 5113 - protein, 9 aa, synthetic construct
GGLGHDTMT

SEQ ID NO: 5114 - protein, 9 aa, synthetic construct
GGAGKDILE

SEQ ID NO: 5115 - protein, 9 aa, synthetic construct
GGLGNDSLN

SEQ ID NO: 5116 - protein, 9 aa, synthetic construct
GGLGSDLIV

SEQ ID NO: 5117 - protein, 9 aa, synthetic construct
GGAGSDRLF

SEQ ID NO: 5118 - protein, 9 aa, synthetic construct
GGNGNDRLN

SEQ ID NO: 5119 - protein, 9 aa, synthetic construct
GGLGDDVIA

SEQ ID NO: 5120 - protein, 9 aa, synthetic construct
GGVGDDTLI

SEQ ID NO: 5121 - protein, 9 aa, synthetic construct
GGAGGDLLI

SEQ ID NO: 5122 - protein, 9 aa, synthetic construct
GGSGADVLS

SEQ ID NO: 5123 - protein, 9 aa, synthetic construct
GGSGADVLV

SEQ ID NO: 5124 - protein, 9 aa, synthetic construct
GGIGNDILI

SEQ ID NO: 5125 - protein, 9 aa, synthetic construct
GGEGNDLLQ

SEQ ID NO: 5126 - protein, 9 aa, synthetic construct
GGYGDDYID

SEQ ID NO: 5127 - protein, 9 aa, synthetic construct
GGNGNDSIL

SEQ ID NO: 5128 - protein, 9 aa, synthetic construct
GGAGDDLIA

SEQ ID NO: 5129 - protein, 9 aa, synthetic construct
GGAGNDTFH

SEQ ID NO: 5130 - protein, 9 aa, synthetic construct
GGDGNDSIE

SEQ ID NO: 5131 - protein, 9 aa, synthetic construct
GGVGDDVLT

SEQ ID NO: 5132 - protein, 9 aa, synthetic construct
GGDGEDTLI

SEQ ID NO: 5133 - protein, 9 aa, synthetic construct
GGNGDDSFD

SEQ ID NO: 5134 - protein, 9 aa, synthetic construct
GGDGDDMIG

SEQ ID NO: 5135 - protein, 9 aa, synthetic construct
GGVGNDVLI

SEQ ID NO: 5136 - protein, 9 aa, synthetic construct
GGTGHDTLA

SEQ ID NO: 5137 - protein, 9 aa, synthetic construct
GGKGADTLN

SEQ ID NO: 5138 - protein, 9 aa, synthetic construct
GGAGDDRVE

SEQ ID NO: 5139 - protein, 9 aa, synthetic construct
GGLGADRME

SEQ ID NO: 5140 - protein, 9 aa, synthetic construct
GGAGNDEID

SEQ ID NO: 5141 - protein, 9 aa, synthetic construct
GGPGDDRLD

SEQ ID NO: 5142 - protein, 9 aa, synthetic construct
GGAGRDVLN

SEQ ID NO: 5143 - protein, 9 aa, synthetic construct
GGIGADTMI

SEQ ID NO: 5144 - protein, 9 aa, synthetic construct
GGGGNDVIV

SEQ ID NO: 5145 - protein, 9 aa, synthetic construct
GGAGADTIA

SEQ ID NO: 5146 - protein, 9 aa, synthetic construct
GGAGDDWIS

SEQ ID NO: 5147 - protein, 9 aa, synthetic construct
GGDGGDRLE

SEQ ID NO: 5148 - protein, 9 aa, synthetic construct
GGAGRDTFA

SEQ ID NO: 5149 - protein, 9 aa, synthetic construct
GGTGDDSLN

SEQ ID NO: 5150 - protein, 9 aa, synthetic construct
GGLGRDVLA

SEQ ID NO: 5151 - protein, 9 aa, synthetic construct
GGSGDDVIL

SEQ ID NO: 5152 - protein, 9 aa, synthetic construct
GGRGNDLLG

SEQ ID NO: 5153 - protein, 9 aa, synthetic construct
GGEGADSLE

SEQ ID NO: 5154 - protein, 9 aa, synthetic construct
GGNGDDLIY

SEQ ID NO: 5155 - protein, 9 aa, synthetic construct
GGAGIDSYH

SEQ ID NO: 5156 - protein, 9 aa, synthetic construct
GGNGADLLA

SEQ ID NO: 5157 - protein, 9 aa, synthetic construct
GGDGIDALF

SEQ ID NO: 5158 - protein, 9 aa, synthetic construct
GGTGDDILR

SEQ ID NO: 5159 - protein, 9 aa, synthetic construct
GGAGRDVLK

SEQ ID NO: 5160 - protein, 9 aa, synthetic construct
GGAGHDRLI

SEQ ID NO: 5161 - protein, 9 aa, synthetic construct
GGTGNDKLL

SEQ ID NO: 5162 - protein, 9 aa, synthetic construct
GGAGRDVLF

SEQ ID NO: 5163 - protein, 9 aa, synthetic construct
GGAGDDVFA

SEQ ID NO: 5164 - protein, 9 aa, synthetic construct
GGDGNDVFV

SEQ ID NO: 5165 - protein, 9 aa, synthetic construct
GGLGNDLIA

SEQ ID NO: 5166 - protein, 9 aa, synthetic construct
GGTGRDRLI

SEQ ID NO: 5167 - protein, 9 aa, synthetic construct
GGGGVDTFV

SEQ ID NO: 5168 - protein, 9 aa, synthetic construct
GGRGNDMLL

SEQ ID NO: 5169 - protein, 9 aa, synthetic construct
GGEGADVLN

SEQ ID NO: 5170 - protein, 9 aa, synthetic construct
GGTGNDTLW

SEQ ID NO: 5171 - protein, 9 aa, synthetic construct
GGTGNDTMA

SEQ ID NO: 5172 - protein, 9 aa, synthetic construct
GGSGDDVIV

SEQ ID NO: 5173 - protein, 9 aa, synthetic construct
GGAGHDRLD

SEQ ID NO: 5174 - protein, 9 aa, synthetic construct
GGTGDDQLS

SEQ ID NO: 5175 - protein, 9 aa, synthetic construct
GGDGNDWLS

SEQ ID NO: 5176 - protein, 9 aa, synthetic construct
GGAGEDSLF

SEQ ID NO: 5177 - protein, 9 aa, synthetic construct
GGLGNDIIY

SEQ ID NO: 5178 - protein, 9 aa, synthetic construct
GGWGNDWIS

SEQ ID NO: 5179 - protein, 9 aa, synthetic construct
GGSGDDVFR

SEQ ID NO: 5180 - protein, 9 aa, synthetic construct
GGAGNDYIV

SEQ ID NO: 5181 - protein, 9 aa, synthetic construct
GGAGRDILF

SEQ ID NO: 5182 - protein, 9 aa, synthetic construct
GGEGDDALY

SEQ ID NO: 5183 - protein, 9 aa, synthetic construct
GGDGNDSMS

SEQ ID NO: 5184 - protein, 9 aa, synthetic construct
GGAGADSMV

SEQ ID NO: 5185 - protein, 9 aa, synthetic construct
GGAGNDYIY

SEQ ID NO: 5186 - protein, 9 aa, synthetic construct
GGEGTDSLT

SEQ ID NO: 5187 - protein, 9 aa, synthetic construct
GGDGEDKIF

SEQ ID NO: 5188 - protein, 9 aa, synthetic construct
GGPGHDSLS

SEQ ID NO: 5189 - protein, 9 aa, synthetic construct
GGTGSDTLS

SEQ ID NO: 5190 - protein, 9 aa, synthetic construct
GGSGSDLLI

SEQ ID NO: 5191 - protein, 9 aa, synthetic construct
GGKGDDVID

SEQ ID NO: 5192 - protein, 9 aa, synthetic construct
GGLGDDFLL

SEQ ID NO: 5193 - protein, 9 aa, synthetic construct
GGAGADELS

SEQ ID NO: 5194 - protein, 9 aa, synthetic construct
GGDGADVIN

SEQ ID NO: 5195 - protein, 9 aa, synthetic construct
GGKGNDRLM

SEQ ID NO: 5196 - protein, 9 aa, synthetic construct
GGAGRDSLV

SEQ ID NO: 5197 - protein, 9 aa, synthetic construct
GGTGDDTIA

SEQ ID NO: 5198 - protein, 9 aa, synthetic construct
GGAGDDSYV

SEQ ID NO: 5199 - protein, 9 aa, synthetic construct
GGDGADVLY

SEQ ID NO: 5200 - protein, 9 aa, synthetic construct
GGDGNDVYV

SEQ ID NO: 5201 - protein, 9 aa, synthetic construct
GGDGADVLF

SEQ ID NO: 5202 - protein, 9 aa, synthetic construct
GGMGDDTLV

SEQ ID NO: 5203 - protein, 9 aa, synthetic construct
GGAGEDSLS

SEQ ID NO: 5204 - protein, 9 aa, synthetic construct
GGAGADTIF

SEQ ID NO: 5205 - protein, 9 aa, synthetic construct
GGFGNDTIE

SEQ ID NO: 5206 - protein, 9 aa, synthetic construct
GGAGADQFR

SEQ ID NO: 5207 - protein, 9 aa, synthetic construct
GGGGADLLS

SEQ ID NO: 5208 - protein, 9 aa, synthetic construct
GGTGNDQLN

SEQ ID NO: 5209 - protein, 9 aa, synthetic construct
GGSGVDTLH

SEQ ID NO: 5210 - protein, 9 aa, synthetic construct
GGRGDDVLE

SEQ ID NO: 5211 - protein, 9 aa, synthetic construct
GGRGNDTAL

SEQ ID NO: 5212 - protein, 9 aa, synthetic construct
GGDGDDLIA

SEQ ID NO: 5213 - protein, 9 aa, synthetic construct
GGTGDDRLF

SEQ ID NO: 5214 - protein, 9 aa, synthetic construct
GGLGADVMS

SEQ ID NO: 5215 - protein, 9 aa, synthetic construct
GGAGADTFS

SEQ ID NO: 5216 - protein, 9 aa, synthetic construct
GGRGDDVLD

SEQ ID NO: 5217 - protein, 9 aa, synthetic construct
GGNGDDILD

SEQ ID NO: 5218 - protein, 9 aa, synthetic construct
GGAGNDNLG

SEQ ID NO: 5219 - protein, 9 aa, synthetic construct
GGDGNDIIT

SEQ ID NO: 5220 - protein, 9 aa, synthetic construct
GGFGNDTLV

SEQ ID NO: 5221 - protein, 9 aa, synthetic construct
GGDGSDTYF

SEQ ID NO: 5222 - protein, 9 aa, synthetic construct
GGEGNDRIY

SEQ ID NO: 5223 - protein, 9 aa, synthetic construct
GGAGEDTLN

SEQ ID NO: 5224 - protein, 9 aa, synthetic construct
GGIGADWLV

SEQ ID NO: 5225 - protein, 9 aa, synthetic construct
GGDGHDVLS

SEQ ID NO: 5226 - protein, 9 aa, synthetic construct
GGRGNDSYV

SEQ ID NO: 5227 - protein, 9 aa, synthetic construct
GGFGYDRLN

SEQ ID NO: 5228 - protein, 9 aa, synthetic construct
GGAGADVLF

SEQ ID NO: 5229 - protein, 9 aa, synthetic construct
GGGGQDVVD

SEQ ID NO: 5230 - protein, 9 aa, synthetic construct
GGDGSDKLF

SEQ ID NO: 5231 - protein, 9 aa, synthetic construct
GGEGDDTYV

SEQ ID NO: 5232 - protein, 9 aa, synthetic construct
GGAGNDALQ

SEQ ID NO: 5233 - protein, 9 aa, synthetic construct
GGDGNDIII

SEQ ID NO: 5234 - protein, 9 aa, synthetic construct
GGAGADVIS

SEQ ID NO: 5235 - protein, 9 aa, synthetic construct
GGAGTDKLT

SEQ ID NO: 5236 - protein, 9 aa, synthetic construct
GGIGDDYLY

SEQ ID NO: 5237 - protein, 9 aa, synthetic construct
GGAGDDTMD

SEQ ID NO: 5238 - protein, 9 aa, synthetic construct
GGDGDDELD

SEQ ID NO: 5239 - protein, 9 aa, synthetic construct
GGAGQDRLL

SEQ ID NO: 5240 - protein, 9 aa, synthetic construct
GGRGADQLY

SEQ ID NO: 5241 - protein, 9 aa, synthetic construct
GGPGDDTLV

SEQ ID NO: 5242 - protein, 9 aa, synthetic construct
GGPGNDILY

SEQ ID NO: 5243 - protein, 9 aa, synthetic construct
GGAGADRMS

SEQ ID NO: 5244 - protein, 9 aa, synthetic construct
GGAGVDTMI

SEQ ID NO: 5245 - protein, 9 aa, synthetic construct
GGTGDDKLF

SEQ ID NO: 5246 - protein, 9 aa, synthetic construct
GGGGADHFV

SEQ ID NO: 5247 - protein, 9 aa, synthetic construct
GGNGNDIYV

SEQ ID NO: 5248 - protein, 9 aa, synthetic construct
GGSGEDTFK

SEQ ID NO: 5249 - protein, 9 aa, synthetic construct
GGAGADVFE

SEQ ID NO: 5250 - protein, 9 aa, synthetic construct
GGDGADTFT

SEQ ID NO: 5251 - protein, 9 aa, synthetic construct
GGYGNDTLY

SEQ ID NO: 5252 - protein, 9 aa, synthetic construct
GGAGVDTMT

SEQ ID NO: 5253 - protein, 9 aa, synthetic construct
GGLGADVLE

SEQ ID NO: 5254 - protein, 9 aa, synthetic construct
GGPGNDLLE

SEQ ID NO: 5255 - protein, 9 aa, synthetic construct
GGTGNDTMV

SEQ ID NO: 5256 - protein, 9 aa, synthetic construct
GGSGEDTFR

SEQ ID NO: 5257 - protein, 9 aa, synthetic construct
GGTGRDTLA

SEQ ID NO: 5258 - protein, 9 aa, synthetic construct
GGLGNDILY

SEQ ID NO: 5259 - protein, 9 aa, synthetic construct
GGSGNDLLA

SEQ ID NO: 5260 - protein, 9 aa, synthetic construct
GGGGNDLIY

SEQ ID NO: 5261 - protein, 9 aa, synthetic construct
GGPGNDEIF

SEQ ID NO: 5262 - protein, 9 aa, synthetic construct
GGDGDDTLK

SEQ ID NO: 5263 - protein, 9 aa, synthetic construct
GGRGDDSLT

SEQ ID NO: 5264 - protein, 9 aa, synthetic construct
GGPGDDILS

SEQ ID NO: 5265 - protein, 9 aa, synthetic construct
GGKGDDALY

SEQ ID NO: 5266 - protein, 9 aa, synthetic construct
GGDGHDSLH

SEQ ID NO: 5267 - protein, 9 aa, synthetic construct
GGSGDDYLS

SEQ ID NO: 5268 - protein, 9 aa, synthetic construct
GGAGADVLQ

SEQ ID NO: 5269 - protein, 9 aa, synthetic construct
GGAGADDLT

SEQ ID NO: 5270 - protein, 9 aa, synthetic construct
GGKGTDTLK

SEQ ID NO: 5271 - protein, 9 aa, synthetic construct
GGWGNDLMN

SEQ ID NO: 5272 - protein, 9 aa, synthetic construct
GGAGNDNLQ

SEQ ID NO: 5273 - protein, 9 aa, synthetic construct
GGGGDDRLT

SEQ ID NO: 5274 - protein, 9 aa, synthetic construct
GGNGDDILV

SEQ ID NO: 5275 - protein, 9 aa, synthetic construct
GGTGNDVVA

SEQ ID NO: 5276 - protein, 9 aa, synthetic construct
GGDGNDTIG

SEQ ID NO: 5277 - protein, 9 aa, synthetic construct
GGMGADRFV

SEQ ID NO: 5278 - protein, 9 aa, synthetic construct
GGNGDDIYR

SEQ ID NO: 5279 - protein, 9 aa, synthetic construct
GGTGDDSID

SEQ ID NO: 5280 - protein, 9 aa, synthetic construct
GGEGNDELF

SEQ ID NO: 5281 - protein, 9 aa, synthetic construct
GGLGNDLLL

SEQ ID NO: 5282 - protein, 9 aa, synthetic construct
GGNGDDRLS

SEQ ID NO: 5283 - protein, 9 aa, synthetic construct
GGIGGDTLD

SEQ ID NO: 5284 - protein, 9 aa, synthetic construct
GGEGADSIL

SEQ ID NO: 5285 - protein, 9 aa, synthetic construct
GGDGDDTVY

SEQ ID NO: 5286 - protein, 9 aa, synthetic construct
GGEGDDRLS

SEQ ID NO: 5287 - protein, 9 aa, synthetic construct
GGKGDDALA

SEQ ID NO: 5288 - protein, 9 aa, synthetic construct
GGKGNDTLE

SEQ ID NO: 5289 - protein, 9 aa, synthetic construct
GGDGDDFLS

SEQ ID NO: 5290 - protein, 9 aa, synthetic construct
GGEGDDTIF

SEQ ID NO: 5291 - protein, 9 aa, synthetic construct
GGEGTDIFV

SEQ ID NO: 5292 - protein, 9 aa, synthetic construct
GGAGHDNIN

SEQ ID NO: 5293 - protein, 9 aa, synthetic construct
GGDGNDFIA

SEQ ID NO: 5294 - protein, 9 aa, synthetic construct
GGEGSDTLK

SEQ ID NO: 5295 - protein, 9 aa, synthetic construct
GGEGDDVIE

SEQ ID NO: 5296 - protein, 9 aa, synthetic construct
GGGGNDTLM

SEQ ID NO: 5297 - protein, 9 aa, synthetic construct
GGIGDDILV

SEQ ID NO: 5298 - protein, 9 aa, synthetic construct
GGEGDDIID

SEQ ID NO: 5299 - protein, 9 aa, synthetic construct
GGAGQDVFV

SEQ ID NO: 5300 - protein, 9 aa, synthetic construct
GGEGADTVS

SEQ ID NO: 5301 - protein, 9 aa, synthetic construct
GGRGDDLLY

SEQ ID NO: 5302 - protein, 9 aa, synthetic construct
GGNGNDLID

SEQ ID NO: 5303 - protein, 9 aa, synthetic construct
GGLGNDFIE

SEQ ID NO: 5304 - protein, 9 aa, synthetic construct
GGGGNDVFI

SEQ ID NO: 5305 - protein, 9 aa, synthetic construct
GGAGSDALD

SEQ ID NO: 5306 - protein, 9 aa, synthetic construct
GGAGEDRLE

SEQ ID NO: 5307 - protein, 9 aa, synthetic construct
GGRGNDVLQ

SEQ ID NO: 5308 - protein, 9 aa, synthetic construct
GGAGNDWID

SEQ ID NO: 5309 - protein, 9 aa, synthetic construct
GGLGADQLT

SEQ ID NO: 5310 - protein, 9 aa, synthetic construct
GGDGNDKLR

SEQ ID NO: 5311 - protein, 9 aa, synthetic construct
GGSGSDILN

SEQ ID NO: 5312 - protein, 9 aa, synthetic construct
GGDGSDQLF

SEQ ID NO: 5313 - protein, 9 aa, synthetic construct
GGAGRDRLL

SEQ ID NO: 5314 - protein, 9 aa, synthetic construct
GGDGDDIIE

SEQ ID NO: 5315 - protein, 9 aa, synthetic construct
GGGGADSID

SEQ ID NO: 5316 - protein, 9 aa, synthetic construct
GGNGIDAAD

SEQ ID NO: 5317 - protein, 9 aa, synthetic construct
GGLGADRLY

SEQ ID NO: 5318 - protein, 9 aa, synthetic construct
GGAGNDVYT

SEQ ID NO: 5319 - protein, 9 aa, synthetic construct
GGRGKDQIL

SEQ ID NO: 5320 - protein, 9 aa, synthetic construct
GGEGNDEIS

SEQ ID NO: 5321 - protein, 9 aa, synthetic construct
GGTGNDELT

SEQ ID NO: 5322 - protein, 9 aa, synthetic construct
GGDGDDGLI

SEQ ID NO: 5323 - protein, 9 aa, synthetic construct
GGGGNDTAS

SEQ ID NO: 5324 - protein, 9 aa, synthetic construct
GGWGNDVLI

SEQ ID NO: 5325 - protein, 9 aa, synthetic construct
GGLGADSLD

SEQ ID NO: 5326 - protein, 9 aa, synthetic construct
GGSGNDLYY

SEQ ID NO: 5327 - protein, 9 aa, synthetic construct
GGTGDDLLR

SEQ ID NO: 5328 - protein, 9 aa, synthetic construct
GGAGYDYAI

SEQ ID NO: 5329 - protein, 9 aa, synthetic construct
GGEGNDQLN

SEQ ID NO: 5330 - protein, 9 aa, synthetic construct
GGKGDDLLN

SEQ ID NO: 5331 - protein, 9 aa, synthetic construct
GGNGGDYIE

SEQ ID NO: 5332 - protein, 9 aa, synthetic construct
GGSGNDFLL

SEQ ID NO: 5333 - protein, 9 aa, synthetic construct
GGTGDDTLH

SEQ ID NO: 5334 - protein, 9 aa, synthetic construct
GGGGYDHYV

SEQ ID NO: 5335 - protein, 9 aa, synthetic construct
GGTGNDSMV

SEQ ID NO: 5336 - protein, 9 aa, synthetic construct
GGRGDDLLR

SEQ ID NO: 5337 - protein, 9 aa, synthetic construct
GGAGNDQID

SEQ ID NO: 5338 - protein, 9 aa, synthetic construct
GGLGADKLI

SEQ ID NO: 5339 - protein, 9 aa, synthetic construct
GGTGADRMQ

SEQ ID NO: 5340 - protein, 9 aa, synthetic construct
GGPGNDRLD

SEQ ID NO: 5341 - protein, 9 aa, synthetic construct
GGAGADDLI

SEQ ID NO: 5342 - protein, 9 aa, synthetic construct
GGNGNDVLF

SEQ ID NO: 5343 - protein, 9 aa, synthetic construct
GGSGSDILV

SEQ ID NO: 5344 - protein, 9 aa, synthetic construct
GGLGRDTLS

SEQ ID NO: 5345 - protein, 9 aa, synthetic construct
GGDGNDIYY

SEQ ID NO: 5346 - protein, 9 aa, synthetic construct
GGSGNDELE

SEQ ID NO: 5347 - protein, 9 aa, synthetic construct
GGRGNDILI

SEQ ID NO: 5348 - protein, 9 aa, synthetic construct
GGEGNDSLN

SEQ ID NO: 5349 - protein, 9 aa, synthetic construct
GGLGNDALT

SEQ ID NO: 5350 - protein, 9 aa, synthetic construct
GGSGDDVFI

SEQ ID NO: 5351 - protein, 9 aa, synthetic construct
GGAGNDYIE

SEQ ID NO: 5352 - protein, 9 aa, synthetic construct
GGDGNDWLM

SEQ ID NO: 5353 - protein, 9 aa, synthetic construct
GGDGVDTLV

SEQ ID NO: 5354 - protein, 9 aa, synthetic construct
GGLGNDELS

SEQ ID NO: 5355 - protein, 9 aa, synthetic construct
GGRGVDRLY

SEQ ID NO: 5356 - protein, 9 aa, synthetic construct
GGLGSDILI

SEQ ID NO: 5357 - protein, 9 aa, synthetic construct
GGAGADTIK

SEQ ID NO: 5358 - protein, 9 aa, synthetic construct
GGLGSDTLY

SEQ ID NO: 5359 - protein, 9 aa, synthetic construct
GGTGDDIID

SEQ ID NO: 5360 - protein, 9 aa, synthetic construct
GGAGADDLD

SEQ ID NO: 5361 - protein, 9 aa, synthetic construct
GGAGLDRMS

SEQ ID NO: 5362 - protein, 9 aa, synthetic construct
GGNGDDTLV

SEQ ID NO: 5363 - protein, 9 aa, synthetic construct
GGKGIDTLI

SEQ ID NO: 5364 - protein, 9 aa, synthetic construct
GGAGNDWLV

SEQ ID NO: 5365 - protein, 9 aa, synthetic construct
GGAGADSFR

SEQ ID NO: 5366 - protein, 9 aa, synthetic construct
GGSGHDVFV

SEQ ID NO: 5367 - protein, 9 aa, synthetic construct
GGNGNDLLQ

SEQ ID NO: 5368 - protein, 9 aa, synthetic construct
GGEGDDILS

SEQ ID NO: 5369 - protein, 9 aa, synthetic construct
GGTGDDIIY

SEQ ID NO: 5370 - protein, 9 aa, synthetic construct
GGRGNDTMT

SEQ ID NO: 5371 - protein, 9 aa, synthetic construct
GGAGRDYLW

SEQ ID NO: 5372 - protein, 9 aa, synthetic construct
GGAGNDMLV

SEQ ID NO: 5373 - protein, 9 aa, synthetic construct
GGLGADTMD

SEQ ID NO: 5374 - protein, 9 aa, synthetic construct
GGAGSDSVI

SEQ ID NO: 5375 - protein, 9 aa, synthetic construct
GGAGSDTMW

SEQ ID NO: 5376 - protein, 9 aa, synthetic construct
GGGGNDILQ

SEQ ID NO: 5377 - protein, 9 aa, synthetic construct
GGEGDDNID

SEQ ID NO: 5378 - protein, 9 aa, synthetic construct
GGDGNDNLL

SEQ ID NO: 5379 - protein, 9 aa, synthetic construct
GGAGLDTLV

SEQ ID NO: 5380 - protein, 9 aa, synthetic construct
GGEGDDELD

SEQ ID NO: 5381 - protein, 9 aa, synthetic construct
GGAGDDWIF

SEQ ID NO: 5382 - protein, 9 aa, synthetic construct
GGGGSDSLY

SEQ ID NO: 5383 - protein, 9 aa, synthetic construct
GGDGADLLT

SEQ ID NO: 5384 - protein, 9 aa, synthetic construct
GGTGNDTVY

SEQ ID NO: 5385 - protein, 9 aa, synthetic construct
GGAGSDTMI

SEQ ID NO: 5386 - protein, 9 aa, synthetic construct
GGAGGDQLV

SEQ ID NO: 5387 - protein, 9 aa, synthetic construct
GGTGSDKLL

SEQ ID NO: 5388 - protein, 9 aa, synthetic construct
GGDGNDNLN

SEQ ID NO: 5389 - protein, 9 aa, synthetic construct
GGRGDDLLE

SEQ ID NO: 5390 - protein, 9 aa, synthetic construct
GGFGNDVLR

SEQ ID NO: 5391 - protein, 9 aa, synthetic construct
GGSGSDKLY

SEQ ID NO: 5392 - protein, 9 aa, synthetic construct
GGSGRDRLD

SEQ ID NO: 5393 - protein, 9 aa, synthetic construct
GGGGNDQLF

SEQ ID NO: 5394 - protein, 9 aa, synthetic construct
GGVGNDTIY

SEQ ID NO: 5395 - protein, 9 aa, synthetic construct
GGRGDDILL

SEQ ID NO: 5396 - protein, 9 aa, synthetic construct
GGTGADLMI

SEQ ID NO: 5397 - protein, 9 aa, synthetic construct
GGSGVDTLI

SEQ ID NO: 5398 - protein, 9 aa, synthetic construct
GGDGADKLY

SEQ ID NO: 5399 - protein, 9 aa, synthetic construct
GGAGADIMR

SEQ ID NO: 5400 - protein, 9 aa, synthetic construct
GGRGNDWLY

SEQ ID NO: 5401 - protein, 9 aa, synthetic construct
GGWGDDSLA

SEQ ID NO: 5402 - protein, 9 aa, synthetic construct
GGTGADSID

SEQ ID NO: 5403 - protein, 9 aa, synthetic construct
GGRGDDTLL

SEQ ID NO: 5404 - protein, 9 aa, synthetic construct
GGVGNDTLQ

SEQ ID NO: 5405 - protein, 9 aa, synthetic construct
GGGGWDTLS

SEQ ID NO: 5406 - protein, 9 aa, synthetic construct
GGIGDDTLL

SEQ ID NO: 5407 - protein, 9 aa, synthetic construct
GGRGDDTLF

SEQ ID NO: 5408 - protein, 9 aa, synthetic construct
GGNGNDMLY

SEQ ID NO: 5409 - protein, 9 aa, synthetic construct
GGEGTDTLN

SEQ ID NO: 5410 - protein, 9 aa, synthetic construct
GGVGNDTLW

SEQ ID NO: 5411 - protein, 9 aa, synthetic construct
GGAGDDYIE

SEQ ID NO: 5412 - protein, 9 aa, synthetic construct
GGAGADTIG

SEQ ID NO: 5413 - protein, 9 aa, synthetic construct
GGAGQDRLD

SEQ ID NO: 5414 - protein, 9 aa, synthetic construct
GGDGADTIF

SEQ ID NO: 5415 - protein, 9 aa, synthetic construct
GGAGADRLH

SEQ ID NO: 5416 - protein, 9 aa, synthetic construct
GGSGDDTII

SEQ ID NO: 5417 - protein, 9 aa, synthetic construct
GGPGDDTLI

SEQ ID NO: 5418 - protein, 9 aa, synthetic construct
GGTGADRLF

SEQ ID NO: 5419 - protein, 9 aa, synthetic construct
GGRGNDTIR

SEQ ID NO: 5420 - protein, 9 aa, synthetic construct
GGTGSDLLT

SEQ ID NO: 5421 - protein, 9 aa, synthetic construct
GGTGDDRLR

SEQ ID NO: 5422 - protein, 9 aa, synthetic construct
GGLGDDVVN

SEQ ID NO: 5423 - protein, 9 aa, synthetic construct
GGIGNDLLF

SEQ ID NO: 5424 - protein, 9 aa, synthetic construct
GGEGADLFV

SEQ ID NO: 5425 - protein, 9 aa, synthetic construct
GGRGNDTLK

SEQ ID NO: 5426 - protein, 9 aa, synthetic construct
GGYGNDNMS

SEQ ID NO: 5427 - protein, 9 aa, synthetic construct
GGEGDDIYI

SEQ ID NO: 5428 - protein, 9 aa, synthetic construct
GGIGDDTVV

SEQ ID NO: 5429 - protein, 9 aa, synthetic construct
GGAGSDTIN

SEQ ID NO: 5430 - protein, 9 aa, synthetic construct
GGEGNDTAV

SEQ ID NO: 5431 - protein, 9 aa, synthetic construct
GGSGSDYLD

SEQ ID NO: 5432 - protein, 9 aa, synthetic construct
GGSGNDILG

SEQ ID NO: 5433 - protein, 9 aa, synthetic construct
GGRGNDVID

SEQ ID NO: 5434 - protein, 9 aa, synthetic construct
GGSGNDVYV

SEQ ID NO: 5435 - protein, 9 aa, synthetic construct
GGGGADFLD

SEQ ID NO: 5436 - protein, 9 aa, synthetic construct
GGSGDDELH

SEQ ID NO: 5437 - protein, 9 aa, synthetic construct
GGAGDDVYK

SEQ ID NO: 5438 - protein, 9 aa, synthetic construct
GGSGVDTLT

SEQ ID NO: 5439 - protein, 9 aa, synthetic construct
GGLGSDTLF

SEQ ID NO: 5440 - protein, 9 aa, synthetic construct
GGAGNDFIQ

SEQ ID NO: 5441 - protein, 9 aa, synthetic construct
GGTGNDTIV

SEQ ID NO: 5442 - protein, 9 aa, synthetic construct
GGAGVDTIT

SEQ ID NO: 5443 - protein, 9 aa, synthetic construct
GGKGDDIII

SEQ ID NO: 5444 - protein, 9 aa, synthetic construct
GGRGNDTYY

SEQ ID NO: 5445 - protein, 9 aa, synthetic construct
GGAGNDSVF

SEQ ID NO: 5446 - protein, 9 aa, synthetic construct
GGSGVDTLS

SEQ ID NO: 5447 - protein, 9 aa, synthetic construct
GGKGNDSLY

SEQ ID NO: 5448 - protein, 9 aa, synthetic construct
GGRGDDRLD

SEQ ID NO: 5449 - protein, 9 aa, synthetic construct
GGIGADTLY

SEQ ID NO: 5450 - protein, 9 aa, synthetic construct
GGAGNDSLK

SEQ ID NO: 5451 - protein, 9 aa, synthetic construct
GGTGNDTFS

SEQ ID NO: 5452 - protein, 9 aa, synthetic construct
GGNGDDFIN

SEQ ID NO: 5453 - protein, 9 aa, synthetic construct
GGEGNDLIE

SEQ ID NO: 5454 - protein, 9 aa, synthetic construct
GGPGDDTLA

SEQ ID NO: 5455 - protein, 9 aa, synthetic construct
GGEGDDTIT

SEQ ID NO: 5456 - protein, 9 aa, synthetic construct
GGSGDDALH

SEQ ID NO: 5457 - protein, 9 aa, synthetic construct
GGGGNDKLV

SEQ ID NO: 5458 - protein, 9 aa, synthetic construct
GGSGNDTVS

SEQ ID NO: 5459 - protein, 9 aa, synthetic construct
GGAGDDILM

SEQ ID NO: 5460 - protein, 9 aa, synthetic construct
GGAGDDIYL

SEQ ID NO: 5461 - protein, 9 aa, synthetic construct
GGTGADAFI

SEQ ID NO: 5462 - protein, 9 aa, synthetic construct
GGDGTDRLS

SEQ ID NO: 5463 - protein, 9 aa, synthetic construct
GGIGADTMT

SEQ ID NO: 5464 - protein, 9 aa, synthetic construct
GGKGADDLY

SEQ ID NO: 5465 - protein, 9 aa, synthetic construct
GGRGDDLLT

SEQ ID NO: 5466 - protein, 9 aa, synthetic construct
GGDGNDDLR

SEQ ID NO: 5467 - protein, 9 aa, synthetic construct
GGRGDDSLD

SEQ ID NO: 5468 - protein, 9 aa, synthetic construct
GGDGADLLF

SEQ ID NO: 5469 - protein, 9 aa, synthetic construct
GGDGDDFIF

SEQ ID NO: 5470 - protein, 9 aa, synthetic construct
GGPGHDRMF

SEQ ID NO: 5471 - protein, 9 aa, synthetic construct
GGVGNDTYL

SEQ ID NO: 5472 - protein, 9 aa, synthetic construct
GGNGSDTLS

SEQ ID NO: 5473 - protein, 9 aa, synthetic construct
GGAGNDSMV

SEQ ID NO: 5474 - protein, 9 aa, synthetic construct
GGDGNDRIL

SEQ ID NO: 5475 - protein, 9 aa, synthetic construct
GGPGHDTLH

SEQ ID NO: 5476 - protein, 9 aa, synthetic construct
GGAGVDTLA

SEQ ID NO: 5477 - protein, 9 aa, synthetic construct
GGNGNDMFY

SEQ ID NO: 5478 - protein, 9 aa, synthetic construct
GGDGNDQLA

SEQ ID NO: 5479 - protein, 9 aa, synthetic construct
GGNGSDTLN

SEQ ID NO: 5480 - protein, 9 aa, synthetic construct
GGKGNDSLS

SEQ ID NO: 5481 - protein, 9 aa, synthetic construct
GGNGSDTLL

SEQ ID NO: 5482 - protein, 9 aa, synthetic construct
GGIGNDLLI

SEQ ID NO: 5483 - protein, 9 aa, synthetic construct
GGAGGDTLY

SEQ ID NO: 5484 - protein, 9 aa, synthetic construct
GGSGNDSLR

SEQ ID NO: 5485 - protein, 9 aa, synthetic construct
GGAGNDRIT

SEQ ID NO: 5486 - protein, 9 aa, synthetic construct
GGAGSDYLS

SEQ ID NO: 5487 - protein, 9 aa, synthetic construct
GGSGNDTFS

SEQ ID NO: 5488 - protein, 9 aa, synthetic construct
GGMGNDSIH

SEQ ID NO: 5489 - protein, 9 aa, synthetic construct
GGHGDDTLL

SEQ ID NO: 5490 - protein, 9 aa, synthetic construct
GGGGNDRMT

SEQ ID NO: 5491 - protein, 9 aa, synthetic construct
GGKGHDSIT

SEQ ID NO: 5492 - protein, 9 aa, synthetic construct
GGNGNDELF

SEQ ID NO: 5493 - protein, 9 aa, synthetic construct
GGSGSDTMT

SEQ ID NO: 5494 - protein, 9 aa, synthetic construct
GGGGIDTAD

SEQ ID NO: 5495 - protein, 9 aa, synthetic construct
GGIGDDILD

SEQ ID NO: 5496 - protein, 9 aa, synthetic construct
GGAGADHFA

SEQ ID NO: 5497 - protein, 9 aa, synthetic construct
GGTGRDILS

SEQ ID NO: 5498 - protein, 9 aa, synthetic construct
GGHGEDTLK

SEQ ID NO: 5499 - protein, 9 aa, synthetic construct
GGGGNDTMF

SEQ ID NO: 5500 - protein, 9 aa, synthetic construct
GGTGEDVLF

SEQ ID NO: 5501 - protein, 9 aa, synthetic construct
GGSGSDTAV

SEQ ID NO: 5502 - protein, 9 aa, synthetic construct
GGVGNDRLL

SEQ ID NO: 5503 - protein, 9 aa, synthetic construct
GGNGDDTVI

SEQ ID NO: 5504 - protein, 9 aa, synthetic construct
GGGGSDMFV

SEQ ID NO: 5505 - protein, 9 aa, synthetic construct
GGGGNDIYI

SEQ ID NO: 5506 - protein, 9 aa, synthetic construct
GGAGKDTMI

SEQ ID NO: 5507 - protein, 9 aa, synthetic construct
GGDGKDTAV

SEQ ID NO: 5508 - protein, 9 aa, synthetic construct
GGTGDDQLF

SEQ ID NO: 5509 - protein, 9 aa, synthetic construct
GGDGDDRIS

SEQ ID NO: 5510 - protein, 9 aa, synthetic construct
GGSGNDEIH

SEQ ID NO: 5511 - protein, 9 aa, synthetic construct
GGAGTDMIQ

SEQ ID NO: 5512 - protein, 9 aa, synthetic construct
GGDGTDTLT

SEQ ID NO: 5513 - protein, 9 aa, synthetic construct
GGNGRDYID

SEQ ID NO: 5514 - protein, 9 aa, synthetic construct
GGAGGDVLS

SEQ ID NO: 5515 - protein, 9 aa, synthetic construct
GGAGADHLS

SEQ ID NO: 5516 - protein, 9 aa, synthetic construct
GGSGDDMLD

SEQ ID NO: 5517 - protein, 9 aa, synthetic construct
GGVGNDALF

SEQ ID NO: 5518 - protein, 9 aa, synthetic construct
GGFGFDTLI

SEQ ID NO: 5519 - protein, 9 aa, synthetic construct
GGDGADVLS

SEQ ID NO: 5520 - protein, 9 aa, synthetic construct
GGTGRDLLV

SEQ ID NO: 5521 - protein, 9 aa, synthetic construct
GGGGSDVLQ

SEQ ID NO: 5522 - protein, 9 aa, synthetic construct
GGIGDDSLL

SEQ ID NO: 5523 - protein, 9 aa, synthetic construct
GGAGRDILS

SEQ ID NO: 5524 - protein, 9 aa, synthetic construct
GGEGNDTYY

SEQ ID NO: 5525 - protein, 9 aa, synthetic construct
GGQGDDLIY

SEQ ID NO: 5526 - protein, 9 aa, synthetic construct
GGGGNDALI

SEQ ID NO: 5527 - protein, 9 aa, synthetic construct
GGDGNDRIF

SEQ ID NO: 5528 - protein, 9 aa, synthetic construct
GGSGDDNLQ

SEQ ID NO: 5529 - protein, 9 aa, synthetic construct
GGAGNDIIA

SEQ ID NO: 5530 - protein, 9 aa, synthetic construct
GGDGDDFIS

SEQ ID NO: 5531 - protein, 9 aa, synthetic construct
GGDGNDRVW

SEQ ID NO: 5532 - protein, 9 aa, synthetic construct
GGIGWDTLR

SEQ ID NO: 5533 - protein, 9 aa, synthetic construct
GGAGDDFID

SEQ ID NO: 5534 - protein, 9 aa, synthetic construct
GGGGDDRIY

SEQ ID NO: 5535 - protein, 9 aa, synthetic construct
GGLGADSLI

SEQ ID NO: 5536 - protein, 9 aa, synthetic construct
GGSGDDRLV

SEQ ID NO: 5537 - protein, 9 aa, synthetic construct
GGVGNDLLY

SEQ ID NO: 5538 - protein, 9 aa, synthetic construct
GGDGNDELT

SEQ ID NO: 5539 - protein, 9 aa, synthetic construct
GGLGADRLF

SEQ ID NO: 5540 - protein, 9 aa, synthetic construct
GGDGSDQLY

SEQ ID NO: 5541 - protein, 9 aa, synthetic construct
GGTGEDGIL

SEQ ID NO: 5542 - protein, 9 aa, synthetic construct
GGLGSDSLY

SEQ ID NO: 5543 - protein, 9 aa, synthetic construct
GGLGADTIN

SEQ ID NO: 5544 - protein, 9 aa, synthetic construct
GGAGEDLVS

SEQ ID NO: 5545 - protein, 9 aa, synthetic construct
GGDGSDQLT

SEQ ID NO: 5546 - protein, 9 aa, synthetic construct
GGKGNDRID

SEQ ID NO: 5547 - protein, 9 aa, synthetic construct
GGGGADILV

SEQ ID NO: 5548 - protein, 9 aa, synthetic construct
GGEGNDSIS

SEQ ID NO: 5549 - protein, 9 aa, synthetic construct
GGLGNDTVF

SEQ ID NO: 5550 - protein, 9 aa, synthetic construct
GGTGQDTID

SEQ ID NO: 5551 - protein, 9 aa, synthetic construct
GGMGNDLLL

SEQ ID NO: 5552 - protein, 9 aa, synthetic construct
GGDGDDLIG

SEQ ID NO: 5553 - protein, 9 aa, synthetic construct
GGEGDDVLK

SEQ ID NO: 5554 - protein, 9 aa, synthetic construct
GGSGEDRLI

SEQ ID NO: 5555 - protein, 9 aa, synthetic construct
GGAGVDYLD

SEQ ID NO: 5556 - protein, 9 aa, synthetic construct
GGDGADQLS

SEQ ID NO: 5557 - protein, 9 aa, synthetic construct
GGAGDDFLF

SEQ ID NO: 5558 - protein, 9 aa, synthetic construct
GGTGQDILA

SEQ ID NO: 5559 - protein, 9 aa, synthetic construct
GGDGDDRII

SEQ ID NO: 5560 - protein, 9 aa, synthetic construct
GGRGNDFLA

SEQ ID NO: 5561 - protein, 9 aa, synthetic construct
GGIGDDILS

SEQ ID NO: 5562 - protein, 9 aa, synthetic construct
GGDGNDEIR

SEQ ID NO: 5563 - protein, 9 aa, synthetic construct
GGSGSDTLN

SEQ ID NO: 5564 - protein, 9 aa, synthetic construct
GGAGQDVLT

SEQ ID NO: 5565 - protein, 9 aa, synthetic construct
GGTGADSLA

SEQ ID NO: 5566 - protein, 9 aa, synthetic construct
GGAGQDVLV

SEQ ID NO: 5567 - protein, 9 aa, synthetic construct
GGEGNDKLH

SEQ ID NO: 5568 - protein, 9 aa, synthetic construct
GGAGKDKLV

SEQ ID NO: 5569 - protein, 9 aa, synthetic construct
GGDGNDELI

SEQ ID NO: 5570 - protein, 9 aa, synthetic construct
GGGGGDTLI

SEQ ID NO: 5571 - protein, 9 aa, synthetic construct
GGLGNDYLN

SEQ ID NO: 5572 - protein, 9 aa, synthetic construct
GGTGADTLQ

SEQ ID NO: 5573 - protein, 9 aa, synthetic construct
GGNGNDSLI

SEQ ID NO: 5574 - protein, 9 aa, synthetic construct
GGEGNDVIY

SEQ ID NO: 5575 - protein, 9 aa, synthetic construct
GGNGNDDIK

SEQ ID NO: 5576 - protein, 9 aa, synthetic construct
GGDGADQFI

SEQ ID NO: 5577 - protein, 9 aa, synthetic construct
GGLGADTMR

SEQ ID NO: 5578 - protein, 9 aa, synthetic construct
GGWGNDILH

SEQ ID NO: 5579 - protein, 9 aa, synthetic construct
GGAGGDTLK

SEQ ID NO: 5580 - protein, 9 aa, synthetic construct
GGEGDDVLT

SEQ ID NO: 5581 - protein, 9 aa, synthetic construct
GGTGRDVFV

SEQ ID NO: 5582 - protein, 9 aa, synthetic construct
GGTGADVMT

SEQ ID NO: 5583 - protein, 9 aa, synthetic construct
GGTGGDRLL

SEQ ID NO: 5584 - protein, 9 aa, synthetic construct
GGLGADLLR

SEQ ID NO: 5585 - protein, 9 aa, synthetic construct
GGDGRDRLD

SEQ ID NO: 5586 - protein, 9 aa, synthetic construct
GGHGNDELR

SEQ ID NO: 5587 - protein, 9 aa, synthetic construct
GGQGDDVLH

SEQ ID NO: 5588 - protein, 9 aa, synthetic construct
GGQGDDVLF

SEQ ID NO: 5589 - protein, 9 aa, synthetic construct
GGSGSDSLS

SEQ ID NO: 5590 - protein, 9 aa, synthetic construct
GGAGIDAVT

SEQ ID NO: 5591 - protein, 9 aa, synthetic construct
GGAGIDRLV

SEQ ID NO: 5592 - protein, 9 aa, synthetic construct
GGAGGDTLR

SEQ ID NO: 5593 - protein, 9 aa, synthetic construct
GGAGADALL

SEQ ID NO: 5594 - protein, 9 aa, synthetic construct
GGEGDDTLG

SEQ ID NO: 5595 - protein, 9 aa, synthetic construct
GGEGDDELY

SEQ ID NO: 5596 - protein, 9 aa, synthetic construct
GGTGRDTLF

SEQ ID NO: 5597 - protein, 9 aa, synthetic construct
GGTGRDTLE

SEQ ID NO: 5598 - protein, 9 aa, synthetic construct
GGDGDDWLS

SEQ ID NO: 5599 - protein, 9 aa, synthetic construct
GGQGDDTYI

SEQ ID NO: 5600 - protein, 9 aa, synthetic construct
GGAGDDIIH

SEQ ID NO: 5601 - protein, 9 aa, synthetic construct
GGKGNDQLF

SEQ ID NO: 5602 - protein, 9 aa, synthetic construct
GGEGDDSIT

SEQ ID NO: 5603 - protein, 9 aa, synthetic construct
GGAGDDIIN

SEQ ID NO: 5604 - protein, 9 aa, synthetic construct
GGGGNDNLD

SEQ ID NO: 5605 - protein, 9 aa, synthetic construct
GGRGDDTLQ

SEQ ID NO: 5606 - protein, 9 aa, synthetic construct
GGTGGDTLI

SEQ ID NO: 5607 - protein, 9 aa, synthetic construct
GGAGDDILG

SEQ ID NO: 5608 - protein, 9 aa, synthetic construct
GGSGEDTLI

SEQ ID NO: 5609 - protein, 9 aa, synthetic construct
GGAGEDTLV

SEQ ID NO: 5610 - protein, 9 aa, synthetic construct
GGDGRDILV

SEQ ID NO: 5611 - protein, 9 aa, synthetic construct
GGSGDDIID

SEQ ID NO: 5612 - protein, 9 aa, synthetic construct
GGPGDDTLW

SEQ ID NO: 5613 - protein, 9 aa, synthetic construct
GGWGDDSLY

SEQ ID NO: 5614 - protein, 9 aa, synthetic construct
GGAGVDTLQ

SEQ ID NO: 5615 - protein, 9 aa, synthetic construct
GGDGADRIS

SEQ ID NO: 5616 - protein, 9 aa, synthetic construct
GGMGNDTLK

SEQ ID NO: 5617 - protein, 9 aa, synthetic construct
GGAGNDALM

SEQ ID NO: 5618 - protein, 9 aa, synthetic construct
GGLGADLLN

SEQ ID NO: 5619 - protein, 9 aa, synthetic construct
GGTGADTLH

SEQ ID NO: 5620 - protein, 9 aa, synthetic construct
GGTGNDVIY

SEQ ID NO: 5621 - protein, 9 aa, synthetic construct
GGAGADRMF

SEQ ID NO: 5622 - protein, 9 aa, synthetic construct
GGIGADVMR

SEQ ID NO: 5623 - protein, 9 aa, synthetic construct
GGAGADTLM

SEQ ID NO: 5624 - protein, 9 aa, synthetic construct
GGDGSDLLT

SEQ ID NO: 5625 - protein, 9 aa, synthetic construct
GGRGNDLFV

SEQ ID NO: 5626 - protein, 9 aa, synthetic construct
GGLGADTYW

SEQ ID NO: 5627 - protein, 9 aa, synthetic construct
GGNGDDTVD

SEQ ID NO: 5628 - protein, 9 aa, synthetic construct
GGAGGDVFV

SEQ ID NO: 5629 - protein, 9 aa, synthetic construct
GGNGADLLE

SEQ ID NO: 5630 - protein, 9 aa, synthetic construct
GGLGNDVVA

SEQ ID NO: 5631 - protein, 9 aa, synthetic construct
GGAGSDVLY

SEQ ID NO: 5632 - protein, 9 aa, synthetic construct
GGMGDDHLY

SEQ ID NO: 5633 - protein, 9 aa, synthetic construct
GGTGFDYLT

SEQ ID NO: 5634 - protein, 9 aa, synthetic construct
GGKGNDRLS

SEQ ID NO: 5635 - protein, 9 aa, synthetic construct
GGNGNDTII

SEQ ID NO: 5636 - protein, 9 aa, synthetic construct
GGAGNDRMY

SEQ ID NO: 5637 - protein, 9 aa, synthetic construct
GGAGNDRYI

SEQ ID NO: 5638 - protein, 9 aa, synthetic construct
GGSGRDIFV

SEQ ID NO: 5639 - protein, 9 aa, synthetic construct
GGIGDDELY

SEQ ID NO: 5640 - protein, 9 aa, synthetic construct
GGRGNDLLR

SEQ ID NO: 5641 - protein, 9 aa, synthetic construct
GGPGDDVLR

SEQ ID NO: 5642 - protein, 9 aa, synthetic construct
GGSGNDSYV

SEQ ID NO: 5643 - protein, 9 aa, synthetic construct
GGSGEDILN

SEQ ID NO: 5644 - protein, 9 aa, synthetic construct
GGEGDDVIS

SEQ ID NO: 5645 - protein, 9 aa, synthetic construct
GGIGNDTLE

SEQ ID NO: 5646 - protein, 9 aa, synthetic construct
GGAGHDELN

SEQ ID NO: 5647 - protein, 9 aa, synthetic construct
GGVGKDVLT

SEQ ID NO: 5648 - protein, 9 aa, synthetic construct
GGEGNDWLT

SEQ ID NO: 5649 - protein, 9 aa, synthetic construct
GGIGNDYLV

SEQ ID NO: 5650 - protein, 9 aa, synthetic construct
GGTGNDWLW

SEQ ID NO: 5651 - protein, 9 aa, synthetic construct
GGAGKDTLL

SEQ ID NO: 5652 - protein, 9 aa, synthetic construct
GGAGEDTLD

SEQ ID NO: 5653 - protein, 9 aa, synthetic construct
GGAGSDVIY

SEQ ID NO: 5654 - protein, 9 aa, synthetic construct
GGLGNDTIA

SEQ ID NO: 5655 - protein, 9 aa, synthetic construct
GGGGNDRLA

SEQ ID NO: 5656 - protein, 9 aa, synthetic construct
GGEGRDILT

SEQ ID NO: 5657 - protein, 9 aa, synthetic construct
GGSGSDSLV

SEQ ID NO: 5658 - protein, 9 aa, synthetic construct
GGKGNDWLY

SEQ ID NO: 5659 - protein, 9 aa, synthetic construct
GGLGEDTIS

SEQ ID NO: 5660 - protein, 9 aa, synthetic construct
GGDGADTLK

SEQ ID NO: 5661 - protein, 9 aa, synthetic construct
GGVGNDTAD

SEQ ID NO: 5662 - protein, 9 aa, synthetic construct
GGSGSDIFR

SEQ ID NO: 5663 - protein, 9 aa, synthetic construct
GGGGNDMLT

SEQ ID NO: 5664 - protein, 9 aa, synthetic construct
GGAGRDLFV

SEQ ID NO: 5665 - protein, 9 aa, synthetic construct
GGGGADLLV

SEQ ID NO: 5666 - protein, 9 aa, synthetic construct
GGQGDDTLN

SEQ ID NO: 5667 - protein, 9 aa, synthetic construct
GGAGNDNLF

SEQ ID NO: 5668 - protein, 9 aa, synthetic construct
GGKGNDQLS

SEQ ID NO: 5669 - protein, 9 aa, synthetic construct
GGSGDDLLH

SEQ ID NO: 5670 - protein, 9 aa, synthetic construct
GGWGNDTYY

SEQ ID NO: 5671 - protein, 9 aa, synthetic construct
GGAGSDFLS

SEQ ID NO: 5672 - protein, 9 aa, synthetic construct
GGTGADIMR

SEQ ID NO: 5673 - protein, 9 aa, synthetic construct
GGKGFDLIY

SEQ ID NO: 5674 - protein, 9 aa, synthetic construct
GGNGNDSIS

SEQ ID NO: 5675 - protein, 9 aa, synthetic construct
GGSGTDRLE

SEQ ID NO: 5676 - protein, 9 aa, synthetic construct
GGTGKDTLI

SEQ ID NO: 5677 - protein, 9 aa, synthetic construct
GGGGDDTLH

SEQ ID NO: 5678 - protein, 9 aa, synthetic construct
GGLGVDTLN

SEQ ID NO: 5679 - protein, 9 aa, synthetic construct
GGLGDDSLS

SEQ ID NO: 5680 - protein, 9 aa, synthetic construct
GGAGDDSIV

SEQ ID NO: 5681 - protein, 9 aa, synthetic construct
GGKGRDTFV

SEQ ID NO: 5682 - protein, 9 aa, synthetic construct
GGDGFDIAG

SEQ ID NO: 5683 - protein, 9 aa, synthetic construct
GGDGADSLI

SEQ ID NO: 5684 - protein, 9 aa, synthetic construct
GGAGRDVFA

SEQ ID NO: 5685 - protein, 9 aa, synthetic construct
GGNGDDLLL

SEQ ID NO: 5686 - protein, 9 aa, synthetic construct
GGVGNDVLV

SEQ ID NO: 5687 - protein, 9 aa, synthetic construct
GGSGSDRFV

SEQ ID NO: 5688 - protein, 9 aa, synthetic construct
GGQGNDRLV

SEQ ID NO: 5689 - protein, 9 aa, synthetic construct
GGSGTDTLS

SEQ ID NO: 5690 - protein, 9 aa, synthetic construct
GGAGHDTLA

SEQ ID NO: 5691 - protein, 9 aa, synthetic construct
GGEGKDTLV

SEQ ID NO: 5692 - protein, 9 aa, synthetic construct
GGAGNDHLH

SEQ ID NO: 5693 - protein, 9 aa, synthetic construct
GGAGADCFV

SEQ ID NO: 5694 - protein, 9 aa, synthetic construct
GGGGNDVLF

SEQ ID NO: 5695 - protein, 9 aa, synthetic construct
GGEGDDSLH

SEQ ID NO: 5696 - protein, 9 aa, synthetic construct
GGEGVDTVY

SEQ ID NO: 5697 - protein, 9 aa, synthetic construct
GGAGNDTVV

SEQ ID NO: 5698 - protein, 9 aa, synthetic construct
GGEGNDNLA

SEQ ID NO: 5699 - protein, 9 aa, synthetic construct
GGDGDDLFV

SEQ ID NO: 5700 - protein, 9 aa, synthetic construct
GGEGDDWLA

SEQ ID NO: 5701 - protein, 9 aa, synthetic construct
GGAGSDLIF

SEQ ID NO: 5702 - protein, 9 aa, synthetic construct
GGAGDDSLH

SEQ ID NO: 5703 - protein, 9 aa, synthetic construct
GGGGRDTLI

SEQ ID NO: 5704 - protein, 9 aa, synthetic construct
GGAGDDNLT

SEQ ID NO: 5705 - protein, 9 aa, synthetic construct
GGAGADVMD

SEQ ID NO: 5706 - protein, 9 aa, synthetic construct
GGSGNDQLR

SEQ ID NO: 5707 - protein, 9 aa, synthetic construct
GGDGADEIY

SEQ ID NO: 5708 - protein, 9 aa, synthetic construct
GGEGNDTIL

SEQ ID NO: 5709 - protein, 9 aa, synthetic construct
GGDGRDVLL

SEQ ID NO: 5710 - protein, 9 aa, synthetic construct
GGQGNDSLS

SEQ ID NO: 5711 - protein, 9 aa, synthetic construct
GGDGNDSIV

SEQ ID NO: 5712 - protein, 9 aa, synthetic construct
GGDGNDILG

SEQ ID NO: 5713 - protein, 9 aa, synthetic construct
GGSGNDLLE

SEQ ID NO: 5714 - protein, 9 aa, synthetic construct
GGGGDDVIY

SEQ ID NO: 5715 - protein, 9 aa, synthetic construct
GGFGNDTYI

SEQ ID NO: 5716 - protein, 9 aa, synthetic construct
GGAGFDTAS

SEQ ID NO: 5717 - protein, 9 aa, synthetic construct
GGAGSDALN

SEQ ID NO: 5718 - protein, 9 aa, synthetic construct
GGRGSDLID

SEQ ID NO: 5719 - protein, 9 aa, synthetic construct
GGGGKDTLI

SEQ ID NO: 5720 - protein, 9 aa, synthetic construct
GGIGSDLFV

SEQ ID NO: 5721 - protein, 9 aa, synthetic construct
GGPGDDILY

SEQ ID NO: 5722 - protein, 9 aa, synthetic construct
GGNGNDRID

SEQ ID NO: 5723 - protein, 9 aa, synthetic construct
GGEGNDTIH

SEQ ID NO: 5724 - protein, 9 aa, synthetic construct
GGSGGDTID

SEQ ID NO: 5725 - protein, 9 aa, synthetic construct
GGEGADSLS

SEQ ID NO: 5726 - protein, 9 aa, synthetic construct
GGTGKDLLI

SEQ ID NO: 5727 - protein, 9 aa, synthetic construct
GGDGDDTVD

SEQ ID NO: 5728 - protein, 9 aa, synthetic construct
GGNGNDSLT

SEQ ID NO: 5729 - protein, 9 aa, synthetic construct
GGMGLDTLL

SEQ ID NO: 5730 - protein, 9 aa, synthetic construct
GGTGNDGLA

SEQ ID NO: 5731 - protein, 9 aa, synthetic construct
GGDGDDYLR

SEQ ID NO: 5732 - protein, 9 aa, synthetic construct
GGAGADNMI

SEQ ID NO: 5733 - protein, 9 aa, synthetic construct
GGTGNDMLD

SEQ ID NO: 5734 - protein, 9 aa, synthetic construct
GGGGDDVLL

SEQ ID NO: 5735 - protein, 9 aa, synthetic construct
GGTGDDVLF

SEQ ID NO: 5736 - protein, 9 aa, synthetic construct
GGLGNDQMW

SEQ ID NO: 5737 - protein, 9 aa, synthetic construct
GGQGNDMLY

SEQ ID NO: 5738 - protein, 9 aa, synthetic construct
GGDGSDIYY

SEQ ID NO: 5739 - protein, 9 aa, synthetic construct
GGVGRDKLI

SEQ ID NO: 5740 - protein, 9 aa, synthetic construct
GGAGNDWLH

SEQ ID NO: 5741 - protein, 9 aa, synthetic construct
GGEGADSLV

SEQ ID NO: 5742 - protein, 9 aa, synthetic construct
GGNGADTLE

SEQ ID NO: 5743 - protein, 9 aa, synthetic construct
GGAGNDTMV

SEQ ID NO: 5744 - protein, 9 aa, synthetic construct
GGAGKDTID

SEQ ID NO: 5745 - protein, 9 aa, synthetic construct
GGDGNDTMN

SEQ ID NO: 5746 - protein, 9 aa, synthetic construct
GGAGRDTYV

SEQ ID NO: 5747 - protein, 9 aa, synthetic construct
GGGGNDSIA

SEQ ID NO: 5748 - protein, 9 aa, synthetic construct
GGDGSDIYV

SEQ ID NO: 5749 - protein, 9 aa, synthetic construct
GGDGDDMIT

SEQ ID NO: 5750 - protein, 9 aa, synthetic construct
GGEGVDILY

SEQ ID NO: 5751 - protein, 9 aa, synthetic construct
GGEGYDFLA

SEQ ID NO: 5752 - protein, 9 aa, synthetic construct
GGSGNDLMT

SEQ ID NO: 5753 - protein, 9 aa, synthetic construct
GGKGDDHLY

SEQ ID NO: 5754 - protein, 9 aa, synthetic construct
GGAGSDLYR

SEQ ID NO: 5755 - protein, 9 aa, synthetic construct
GGLGNDQLT

SEQ ID NO: 5756 - protein, 9 aa, synthetic construct
GGAGADFIN

SEQ ID NO: 5757 - protein, 9 aa, synthetic construct
GGDGADELR

SEQ ID NO: 5758 - protein, 9 aa, synthetic construct
GGGGDDILA

SEQ ID NO: 5759 - protein, 9 aa, synthetic construct
GGAGSDLID

SEQ ID NO: 5760 - protein, 9 aa, synthetic construct
GGNGDDIIQ

SEQ ID NO: 5761 - protein, 9 aa, synthetic construct
GGSGNDLID

SEQ ID NO: 5762 - protein, 9 aa, synthetic construct
GGTGTDTLI

SEQ ID NO: 5763 - protein, 9 aa, synthetic construct
GGTGDDILE

SEQ ID NO: 5764 - protein, 9 aa, synthetic construct
GGDGNDLIF

SEQ ID NO: 5765 - protein, 9 aa, synthetic construct
GGSGADLLR

SEQ ID NO: 5766 - protein, 9 aa, synthetic construct
GGGGADTII

SEQ ID NO: 5767 - protein, 9 aa, synthetic construct
GGLGKDILT

SEQ ID NO: 5768 - protein, 9 aa, synthetic construct
GGSGNDNLL

SEQ ID NO: 5769 - protein, 9 aa, synthetic construct
GGPGADILT

SEQ ID NO: 5770 - protein, 9 aa, synthetic construct
GGTGDDTYF

SEQ ID NO: 5771 - protein, 9 aa, synthetic construct
GGSGADLLW

SEQ ID NO: 5772 - protein, 9 aa, synthetic construct
GGEGNDYLF

SEQ ID NO: 5773 - protein, 9 aa, synthetic construct
GGKGSDTLV

SEQ ID NO: 5774 - protein, 9 aa, synthetic construct
GGHGADTLS

SEQ ID NO: 5775 - protein, 9 aa, synthetic construct
GGLGNDLIV

SEQ ID NO: 5776 - protein, 9 aa, synthetic construct
GGLGNDVIH

SEQ ID NO: 5777 - protein, 9 aa, synthetic construct
GGAGADVMV

SEQ ID NO: 5778 - protein, 9 aa, synthetic construct
GGEGNDFLD

SEQ ID NO: 5779 - protein, 9 aa, synthetic construct
GGNGGDHLF

SEQ ID NO: 5780 - protein, 9 aa, synthetic construct
GGSGSDQLT

SEQ ID NO: 5781 - protein, 9 aa, synthetic construct
GGEGRDVLR

SEQ ID NO: 5782 - protein, 9 aa, synthetic construct
GGAGADYME

SEQ ID NO: 5783 - protein, 9 aa, synthetic construct
GGPGNDRLQ

SEQ ID NO: 5784 - protein, 9 aa, synthetic construct
GGDGADSFV

SEQ ID NO: 5785 - protein, 9 aa, synthetic construct
GGAGKDALW

SEQ ID NO: 5786 - protein, 9 aa, synthetic construct
GGIGADILI

SEQ ID NO: 5787 - protein, 9 aa, synthetic construct
GGFGNDQMW

SEQ ID NO: 5788 - protein, 9 aa, synthetic construct
GGTGNDIIN

SEQ ID NO: 5789 - protein, 9 aa, synthetic construct
GGNGDDYLH

SEQ ID NO: 5790 - protein, 9 aa, synthetic construct
GGKGSDTYI

SEQ ID NO: 5791 - protein, 9 aa, synthetic construct
GGTGADRLS

SEQ ID NO: 5792 - protein, 9 aa, synthetic construct
GGVGADQLT

SEQ ID NO: 5793 - protein, 9 aa, synthetic construct
GGGGADTIL

SEQ ID NO: 5794 - protein, 9 aa, synthetic construct
GGDGDDSII

SEQ ID NO: 5795 - protein, 9 aa, synthetic construct
GGAGNDVFT

SEQ ID NO: 5796 - protein, 9 aa, synthetic construct
GGTGDDTVT

SEQ ID NO: 5797 - protein, 9 aa, synthetic construct
GGDGDDVFV

SEQ ID NO: 5798 - protein, 9 aa, synthetic construct
GGRGVDFIE

SEQ ID NO: 5799 - protein, 9 aa, synthetic construct
GGLGDDRLT

SEQ ID NO: 5800 - protein, 9 aa, synthetic construct
GGDGLDTLS

SEQ ID NO: 5801 - protein, 9 aa, synthetic construct
GGYGADTLT

SEQ ID NO: 5802 - protein, 9 aa, synthetic construct
GGGGSDTLF

SEQ ID NO: 5803 - protein, 9 aa, synthetic construct
GGTGDDTII

SEQ ID NO: 5804 - protein, 9 aa, synthetic construct
GGDGADVID

SEQ ID NO: 5805 - protein, 9 aa, synthetic construct
GGDGMDRLD

SEQ ID NO: 5806 - protein, 9 aa, synthetic construct
GGTGDDTYL

SEQ ID NO: 5807 - protein, 9 aa, synthetic construct
GGEGADKLV

SEQ ID NO: 5808 - protein, 9 aa, synthetic construct
GGEGDDLIV

SEQ ID NO: 5809 - protein, 9 aa, synthetic construct
GGEGDDVME

SEQ ID NO: 5810 - protein, 9 aa, synthetic construct
GGDGADRVL

SEQ ID NO: 5811 - protein, 9 aa, synthetic construct
GGGGTDTAV

SEQ ID NO: 5812 - protein, 9 aa, synthetic construct
GGGGRDTLL

SEQ ID NO: 5813 - protein, 9 aa, synthetic construct
GGNGNDHLY

SEQ ID NO: 5814 - protein, 9 aa, synthetic construct
GGTGNDKLT

SEQ ID NO: 5815 - protein, 9 aa, synthetic construct
GGEGRDLVD

SEQ ID NO: 5816 - protein, 9 aa, synthetic construct
GGGGADTLQ

SEQ ID NO: 5817 - protein, 9 aa, synthetic construct
GGSGQDRLM

SEQ ID NO: 5818 - protein, 9 aa, synthetic construct
GGGGNDSIL

SEQ ID NO: 5819 - protein, 9 aa, synthetic construct
GGHGRDQLA

SEQ ID NO: 5820 - protein, 9 aa, synthetic construct
GGNGFDRLF

SEQ ID NO: 5821 - protein, 9 aa, synthetic construct
GGEGADRLF

SEQ ID NO: 5822 - protein, 9 aa, synthetic construct
GGAGRDVIL

SEQ ID NO: 5823 - protein, 9 aa, synthetic construct
GGDGDDIAN

SEQ ID NO: 5824 - protein, 9 aa, synthetic construct
GGKGDDTIY

SEQ ID NO: 5825 - protein, 9 aa, synthetic construct
GGTGKDVLL

SEQ ID NO: 5826 - protein, 9 aa, synthetic construct
GGSGADQLF

SEQ ID NO: 5827 - protein, 9 aa, synthetic construct
GGRGSDVLI

SEQ ID NO: 5828 - protein, 9 aa, synthetic construct
GGDGLDTLL

SEQ ID NO: 5829 - protein, 9 aa, synthetic construct
GGVGSDTYV

SEQ ID NO: 5830 - protein, 9 aa, synthetic construct
GGAGSDILF

SEQ ID NO: 5831 - protein, 9 aa, synthetic construct
GGDGDDYLT

SEQ ID NO: 5832 - protein, 9 aa, synthetic construct
GGLGSDTLS

SEQ ID NO: 5833 - protein, 9 aa, synthetic construct
GGKGSDTLI

SEQ ID NO: 5834 - protein, 9 aa, synthetic construct
GGAGNDYMA

SEQ ID NO: 5835 - protein, 9 aa, synthetic construct
GGPGADHLW

SEQ ID NO: 5836 - protein, 9 aa, synthetic construct
GGIGTDTLI

SEQ ID NO: 5837 - protein, 9 aa, synthetic construct
GGKGNDTLK

SEQ ID NO: 5838 - protein, 9 aa, synthetic construct
GGMGADTLI

SEQ ID NO: 5839 - protein, 9 aa, synthetic construct
GGKGSDVLI

SEQ ID NO: 5840 - protein, 9 aa, synthetic construct
GGAGVDLLI

SEQ ID NO: 5841 - protein, 9 aa, synthetic construct
GGPGNDYMD

SEQ ID NO: 5842 - protein, 9 aa, synthetic construct
GGAGDDQIG

SEQ ID NO: 5843 - protein, 9 aa, synthetic construct
GGAGADLMT

SEQ ID NO: 5844 - protein, 9 aa, synthetic construct
GGAGRDVLV

SEQ ID NO: 5845 - protein, 9 aa, synthetic construct
GGDGNDYLR

SEQ ID NO: 5846 - protein, 9 aa, synthetic construct
GGNGADQLI

SEQ ID NO: 5847 - protein, 9 aa, synthetic construct
GGSGNDVLH

SEQ ID NO: 5848 - protein, 9 aa, synthetic construct
GGAGDDTMI

SEQ ID NO: 5849 - protein, 9 aa, synthetic construct
GGQGNDLLY

SEQ ID NO: 5850 - protein, 9 aa, synthetic construct
GGLGDDQLF

SEQ ID NO: 5851 - protein, 9 aa, synthetic construct
GGAGSDDIK

SEQ ID NO: 5852 - protein, 9 aa, synthetic construct
GGYGNDVLI

SEQ ID NO: 5853 - protein, 9 aa, synthetic construct
GGDGIDNLF

SEQ ID NO: 5854 - protein, 9 aa, synthetic construct
GGSGNDIYY

SEQ ID NO: 5855 - protein, 9 aa, synthetic construct
GGGGDDNLS

SEQ ID NO: 5856 - protein, 9 aa, synthetic construct
GGDGADRLN

SEQ ID NO: 5857 - protein, 9 aa, synthetic construct
GGAGADAMI

SEQ ID NO: 5858 - protein, 9 aa, synthetic construct
GGLGDDEMY

SEQ ID NO: 5859 - protein, 9 aa, synthetic construct
GGAGHDSLE

SEQ ID NO: 5860 - protein, 9 aa, synthetic construct
GGAGADKFV

SEQ ID NO: 5861 - protein, 9 aa, synthetic construct
GGGGNDRIF

SEQ ID NO: 5862 - protein, 9 aa, synthetic construct
GGPGNDTID

SEQ ID NO: 5863 - protein, 9 aa, synthetic construct
GGKGNDHLH

SEQ ID NO: 5864 - protein, 9 aa, synthetic construct
GGEGADILQ

SEQ ID NO: 5865 - protein, 9 aa, synthetic construct
GGFGDDTLL

SEQ ID NO: 5866 - protein, 9 aa, synthetic construct
GGAGMDSLS

SEQ ID NO: 5867 - protein, 9 aa, synthetic construct
GGAGSDRLS

SEQ ID NO: 5868 - protein, 9 aa, synthetic construct
GGPGSDRML

SEQ ID NO: 5869 - protein, 9 aa, synthetic construct
GGEGDDILT

SEQ ID NO: 5870 - protein, 9 aa, synthetic construct
GGLGNDSIG

SEQ ID NO: 5871 - protein, 9 aa, synthetic construct
GGLGADEIH

SEQ ID NO: 5872 - protein, 9 aa, synthetic construct
GGDGNDVIE

SEQ ID NO: 5873 - protein, 9 aa, synthetic construct
GGPGADTLF

SEQ ID NO: 5874 - protein, 9 aa, synthetic construct
GGVGDDSLS

SEQ ID NO: 5875 - protein, 9 aa, synthetic construct
GGIGQDTLS

SEQ ID NO: 5876 - protein, 9 aa, synthetic construct
GGAGNDLIQ

SEQ ID NO: 5877 - protein, 9 aa, synthetic construct
GGSGGDTVD

SEQ ID NO: 5878 - protein, 9 aa, synthetic construct
GGVGDDSIL

SEQ ID NO: 5879 - protein, 9 aa, synthetic construct
GGSGNDTYF

SEQ ID NO: 5880 - protein, 9 aa, synthetic construct
GGAGADLIG

SEQ ID NO: 5881 - protein, 9 aa, synthetic construct
GGQGNDALT

SEQ ID NO: 5882 - protein, 9 aa, synthetic construct
GGSGADDLT

SEQ ID NO: 5883 - protein, 9 aa, synthetic construct
GGDGADILI

SEQ ID NO: 5884 - protein, 9 aa, synthetic construct
GGPGKDTFV

SEQ ID NO: 5885 - protein, 9 aa, synthetic construct
GGDGDDLMF

SEQ ID NO: 5886 - protein, 9 aa, synthetic construct
GGAGGDKLN

SEQ ID NO: 5887 - protein, 9 aa, synthetic construct
GGTGSDTLY

SEQ ID NO: 5888 - protein, 9 aa, synthetic construct
GGDGDDIIN

SEQ ID NO: 5889 - protein, 9 aa, synthetic construct
GGAGADTVT

SEQ ID NO: 5890 - protein, 9 aa, synthetic construct
GGDGVDTFR

SEQ ID NO: 5891 - protein, 9 aa, synthetic construct
GGAGTDTIE

SEQ ID NO: 5892 - protein, 9 aa, synthetic construct
GGQGSDSLY

SEQ ID NO: 5893 - protein, 9 aa, synthetic construct
GGLGTDVLT

SEQ ID NO: 5894 - protein, 9 aa, synthetic construct
GGAGIDTLF

SEQ ID NO: 5895 - protein, 9 aa, synthetic construct
GGVGDDTLY

SEQ ID NO: 5896 - protein, 9 aa, synthetic construct
GGFGNDRLF

SEQ ID NO: 5897 - protein, 9 aa, synthetic construct
GGGGEDVLF

SEQ ID NO: 5898 - protein, 9 aa, synthetic construct
GGAGRDRLV

SEQ ID NO: 5899 - protein, 9 aa, synthetic construct
GGIGNDILL

SEQ ID NO: 5900 - protein, 9 aa, synthetic construct
GGPGSDTLL

SEQ ID NO: 5901 - protein, 9 aa, synthetic construct
GGDGIDVLD

SEQ ID NO: 5902 - protein, 9 aa, synthetic construct
GGAGADTME

SEQ ID NO: 5903 - protein, 9 aa, synthetic construct
GGTGADALS

SEQ ID NO: 5904 - protein, 9 aa, synthetic construct
GGDGSDTLF

SEQ ID NO: 5905 - protein, 9 aa, synthetic construct
GGAGNDLII

SEQ ID NO: 5906 - protein, 9 aa, synthetic construct
GGTGNDELI

SEQ ID NO: 5907 - protein, 9 aa, synthetic construct
GGAGSDSFL

SEQ ID NO: 5908 - protein, 9 aa, synthetic construct
GGTGSDRLN

SEQ ID NO: 5909 - protein, 9 aa, synthetic construct
GGKGADKLY

SEQ ID NO: 5910 - protein, 9 aa, synthetic construct
GGAGDDVLW

SEQ ID NO: 5911 - protein, 9 aa, synthetic construct
GGKGSDLLD

SEQ ID NO: 5912 - protein, 9 aa, synthetic construct
GGAGRDRLK

SEQ ID NO: 5913 - protein, 9 aa, synthetic construct
GGGGNDGLS

SEQ ID NO: 5914 - protein, 9 aa, synthetic construct
GGDGSDTIT

SEQ ID NO: 5915 - protein, 9 aa, synthetic construct
GGDGDDTLW

SEQ ID NO: 5916 - protein, 9 aa, synthetic construct
GGAGSDELN

SEQ ID NO: 5917 - protein, 9 aa, synthetic construct
GGDGADTIR

SEQ ID NO: 5918 - protein, 9 aa, synthetic construct
GGSGNDVIL

SEQ ID NO: 5919 - protein, 9 aa, synthetic construct
GGIGNDIIS

SEQ ID NO: 5920 - protein, 9 aa, synthetic construct
GGEGNDILW

SEQ ID NO: 5921 - protein, 9 aa, synthetic construct
GGSGADVLT

SEQ ID NO: 5922 - protein, 9 aa, synthetic construct
GGGGDDLLA

SEQ ID NO: 5923 - protein, 9 aa, synthetic construct
GGEGNDQLD

SEQ ID NO: 5924 - protein, 9 aa, synthetic construct
GGTGADTII

SEQ ID NO: 5925 - protein, 9 aa, synthetic construct
GGKGNDALY

SEQ ID NO: 5926 - protein, 9 aa, synthetic construct
GGTGSDSLY

SEQ ID NO: 5927 - protein, 9 aa, synthetic construct
GGDGDDNLT

SEQ ID NO: 5928 - protein, 9 aa, synthetic construct
GGGGNDWMN

SEQ ID NO: 5929 - protein, 9 aa, synthetic construct
GGNGDDLLV

SEQ ID NO: 5930 - protein, 9 aa, synthetic construct
GGTGNDRVS

SEQ ID NO: 5931 - protein, 9 aa, synthetic construct
GGPGNDTIN

SEQ ID NO: 5932 - protein, 9 aa, synthetic construct
GGFGDDTLN

SEQ ID NO: 5933 - protein, 9 aa, synthetic construct
GGLGDDVIY

SEQ ID NO: 5934 - protein, 9 aa, synthetic construct
GGAGNDVVS

SEQ ID NO: 5935 - protein, 9 aa, synthetic construct
GGNGNDTLH

SEQ ID NO: 5936 - protein, 9 aa, synthetic construct
GGEGADILN

SEQ ID NO: 5937 - protein, 9 aa, synthetic construct
GGAGDDLLW

SEQ ID NO: 5938 - protein, 9 aa, synthetic construct
GGAGADKLA

SEQ ID NO: 5939 - protein, 9 aa, synthetic construct
GGPGNDVLD

SEQ ID NO: 5940 - protein, 9 aa, synthetic construct
GGVGQDTLT

SEQ ID NO: 5941 - protein, 9 aa, synthetic construct
GGRGADRMS

SEQ ID NO: 5942 - protein, 9 aa, synthetic construct
GGAGKDFIV

SEQ ID NO: 5943 - protein, 9 aa, synthetic construct
GGLGNDRIT

SEQ ID NO: 5944 - protein, 9 aa, synthetic construct
GGAGTDVAV

SEQ ID NO: 5945 - protein, 9 aa, synthetic construct
GGDGIDTLD

SEQ ID NO: 5946 - protein, 9 aa, synthetic construct
GGTGNDALN

SEQ ID NO: 5947 - protein, 9 aa, synthetic construct
GGFGDDVLV

SEQ ID NO: 5948 - protein, 9 aa, synthetic construct
GGAGQDALF

SEQ ID NO: 5949 - protein, 9 aa, synthetic construct
GGQGNDILY

SEQ ID NO: 5950 - protein, 9 aa, synthetic construct
GGDGDDSIS

SEQ ID NO: 5951 - protein, 9 aa, synthetic construct
GGTGADFMS

SEQ ID NO: 5952 - protein, 9 aa, synthetic construct
GGEGGDRLY

SEQ ID NO: 5953 - protein, 9 aa, synthetic construct
GGAGGDIFV

SEQ ID NO: 5954 - protein, 9 aa, synthetic construct
GGAGADQLW

SEQ ID NO: 5955 - protein, 9 aa, synthetic construct
GGNGDDTLY

SEQ ID NO: 5956 - protein, 9 aa, synthetic construct
GGKGNDTLA

SEQ ID NO: 5957 - protein, 9 aa, synthetic construct
GGSGNDKLV

SEQ ID NO: 5958 - protein, 9 aa, synthetic construct
GGRGRDTLI

SEQ ID NO: 5959 - protein, 9 aa, synthetic construct
GGAGHDRLW

SEQ ID NO: 5960 - protein, 9 aa, synthetic construct
GGGGQDQLY

SEQ ID NO: 5961 - protein, 9 aa, synthetic construct
GGAGADVIA

SEQ ID NO: 5962 - protein, 9 aa, synthetic construct
GGAGDDTVI

SEQ ID NO: 5963 - protein, 9 aa, synthetic construct
GGGGIDTLN

SEQ ID NO: 5964 - protein, 9 aa, synthetic construct
GGAGADQLR

SEQ ID NO: 5965 - protein, 9 aa, synthetic construct
GGAGYDVLS

SEQ ID NO: 5966 - protein, 9 aa, synthetic construct
GGSGGDTIY

SEQ ID NO: 5967 - protein, 9 aa, synthetic construct
GGSGNDLIA

SEQ ID NO: 5968 - protein, 9 aa, synthetic construct
GGNGNDVLT

SEQ ID NO: 5969 - protein, 9 aa, synthetic construct
GGAGDDRFY

SEQ ID NO: 5970 - protein, 9 aa, synthetic construct
GGEGYDLMR

SEQ ID NO: 5971 - protein, 9 aa, synthetic construct
GGSGRDSLL

SEQ ID NO: 5972 - protein, 9 aa, synthetic construct
GGKGNDLLK

SEQ ID NO: 5973 - protein, 9 aa, synthetic construct
GGKGGDLLD

SEQ ID NO: 5974 - protein, 9 aa, synthetic construct
GGAGDDRIA

SEQ ID NO: 5975 - protein, 9 aa, synthetic construct
GGRGADRLA

SEQ ID NO: 5976 - protein, 9 aa, synthetic construct
GGSGNDLFY

SEQ ID NO: 5977 - protein, 9 aa, synthetic construct
GGEGRDTLI

SEQ ID NO: 5978 - protein, 9 aa, synthetic construct
GGTGKDFLT

SEQ ID NO: 5979 - protein, 9 aa, synthetic construct
GGAGNDLLW

SEQ ID NO: 5980 - protein, 9 aa, synthetic construct
GGAGDDTVE

SEQ ID NO: 5981 - protein, 9 aa, synthetic construct
GGGGNDLLF

SEQ ID NO: 5982 - protein, 9 aa, synthetic construct
GGTGTDELS

SEQ ID NO: 5983 - protein, 9 aa, synthetic construct
GGQGNDILN

SEQ ID NO: 5984 - protein, 9 aa, synthetic construct
GGQGNDILF

SEQ ID NO: 5985 - protein, 9 aa, synthetic construct
GGVGSDLVS

SEQ ID NO: 5986 - protein, 9 aa, synthetic construct
GGAGDDLVA

SEQ ID NO: 5987 - protein, 9 aa, synthetic construct
GGSGADILI

SEQ ID NO: 5988 - protein, 9 aa, synthetic construct
GGAGGDILN

SEQ ID NO: 5989 - protein, 9 aa, synthetic construct
GGAGDDLVR

SEQ ID NO: 5990 - protein, 9 aa, synthetic construct
GGGGQDQYL

SEQ ID NO: 5991 - protein, 9 aa, synthetic construct
GGSGADTLK

SEQ ID NO: 5992 - protein, 9 aa, synthetic construct
GGSGTDILY

SEQ ID NO: 5993 - protein, 9 aa, synthetic construct
GGTGNDQLS

SEQ ID NO: 5994 - protein, 9 aa, synthetic construct
GGPGNDAID

SEQ ID NO: 5995 - protein, 9 aa, synthetic construct
GGAGADAMN

SEQ ID NO: 5996 - protein, 9 aa, synthetic construct
GGRGADTLR

SEQ ID NO: 5997 - protein, 9 aa, synthetic construct
GGAGDDLML

SEQ ID NO: 5998 - protein, 9 aa, synthetic construct
GGSGDDTLH

SEQ ID NO: 5999 - protein, 9 aa, synthetic construct
GGGGNDLIL

SEQ ID NO: 6000 - protein, 9 aa, synthetic construct
GGDGDDELQ

SEQ ID NO: 6001 - protein, 9 aa, synthetic construct
GGDGNDHLI

SEQ ID NO: 6002 - protein, 9 aa, synthetic construct
GGTGSDVLI

SEQ ID NO: 6003 - protein, 9 aa, synthetic construct
GGAGADKLF

SEQ ID NO: 6004 - protein, 9 aa, synthetic construct
GGTGVDTLT

SEQ ID NO: 6005 - protein, 9 aa, synthetic construct
GGDGADSLA

SEQ ID NO: 6006 - protein, 9 aa, synthetic construct
GGYGADTLI

SEQ ID NO: 6007 - protein, 9 aa, synthetic construct
GGDGDDQLE

SEQ ID NO: 6008 - protein, 9 aa, synthetic construct
GGQGSDTLY

SEQ ID NO: 6009 - protein, 9 aa, synthetic construct
GGTGADKLL

SEQ ID NO: 6010 - protein, 9 aa, synthetic construct
GGAGTDTVV

SEQ ID NO: 6011 - protein, 9 aa, synthetic construct
GGKGDDTLF

SEQ ID NO: 6012 - protein, 9 aa, synthetic construct
GGEGEDTLF

SEQ ID NO: 6013 - protein, 9 aa, synthetic construct
GGSGADALD

SEQ ID NO: 6014 - protein, 9 aa, synthetic construct
GGSGADTLF

SEQ ID NO: 6015 - protein, 9 aa, synthetic construct
GGSGDDSLH

SEQ ID NO: 6016 - protein, 9 aa, synthetic construct
GGKGNDELI

SEQ ID NO: 6017 - protein, 9 aa, synthetic construct
GGYGSDKID

SEQ ID NO: 6018 - protein, 9 aa, synthetic construct
GGSGHDRLN

SEQ ID NO: 6019 - protein, 9 aa, synthetic construct
GGTGADTMY

SEQ ID NO: 6020 - protein, 9 aa, synthetic construct
GGGGNDVFE

SEQ ID NO: 6021 - protein, 9 aa, synthetic construct
GGDGNDQMF

SEQ ID NO: 6022 - protein, 9 aa, synthetic construct
GGTGDDTMD

SEQ ID NO: 6023 - protein, 9 aa, synthetic construct
GGNGNDYIG

SEQ ID NO: 6024 - protein, 9 aa, synthetic construct
GGKGNDTYS

SEQ ID NO: 6025 - protein, 9 aa, synthetic construct
GGSGHDTLT

SEQ ID NO: 6026 - protein, 9 aa, synthetic construct
GGKGDDLLD

SEQ ID NO: 6027 - protein, 9 aa, synthetic construct
GGSGRDELY

SEQ ID NO: 6028 - protein, 9 aa, synthetic construct
GGAGNDIIE

SEQ ID NO: 6029 - protein, 9 aa, synthetic construct
GGLGNDVLE

SEQ ID NO: 6030 - protein, 9 aa, synthetic construct
GGAGHDVMR

SEQ ID NO: 6031 - protein, 9 aa, synthetic construct
GGGGGDRLD

SEQ ID NO: 6032 - protein, 9 aa, synthetic construct
GGGGNDVFA

SEQ ID NO: 6033 - protein, 9 aa, synthetic construct
GGAGNDKMS

SEQ ID NO: 6034 - protein, 9 aa, synthetic construct
GGKGNDKLS

SEQ ID NO: 6035 - protein, 9 aa, synthetic construct
GGKGDDILR

SEQ ID NO: 6036 - protein, 9 aa, synthetic construct
GGDGNDQID

SEQ ID NO: 6037 - protein, 9 aa, synthetic construct
GGLGNDYID

SEQ ID NO: 6038 - protein, 9 aa, synthetic construct
GGEGNDIFV

SEQ ID NO: 6039 - protein, 9 aa, synthetic construct
GGSGRDKLY

SEQ ID NO: 6040 - protein, 9 aa, synthetic construct
GGGGNDTVL

SEQ ID NO: 6041 - protein, 9 aa, synthetic construct
GGAGNDIIL

SEQ ID NO: 6042 - protein, 9 aa, synthetic construct
GGTGDDLID

SEQ ID NO: 6043 - protein, 9 aa, synthetic construct
GGAGNDQMH

SEQ ID NO: 6044 - protein, 9 aa, synthetic construct
GGLGNDVLQ

SEQ ID NO: 6045 - protein, 9 aa, synthetic construct
GGAGNDIMS

SEQ ID NO: 6046 - protein, 9 aa, synthetic construct
GGAGHDLIY

SEQ ID NO: 6047 - protein, 9 aa, synthetic construct
GGTGADSMV

SEQ ID NO: 6048 - protein, 9 aa, synthetic construct
GGLGNDVLM

SEQ ID NO: 6049 - protein, 9 aa, synthetic construct
GGAGHDTLV

SEQ ID NO: 6050 - protein, 9 aa, synthetic construct
GGAGHDRLE

SEQ ID NO: 6051 - protein, 9 aa, synthetic construct
GGSGHDHLF

SEQ ID NO: 6052 - protein, 9 aa, synthetic construct
GGTGDDALY

SEQ ID NO: 6053 - protein, 9 aa, synthetic construct
GGFGDDFIE

SEQ ID NO: 6054 - protein, 9 aa, synthetic construct
GGYGNDRIS

SEQ ID NO: 6055 - protein, 9 aa, synthetic construct
GGFGDDLLD

SEQ ID NO: 6056 - protein, 9 aa, synthetic construct
GGTGADSFV

SEQ ID NO: 6057 - protein, 9 aa, synthetic construct
GGLGNDVLL

SEQ ID NO: 6058 - protein, 9 aa, synthetic construct
GGAGNDIMH

SEQ ID NO: 6059 - protein, 9 aa, synthetic construct
GGGGNDVFV

SEQ ID NO: 6060 - protein, 9 aa, synthetic construct
GGSGDDTLK

SEQ ID NO: 6061 - protein, 9 aa, synthetic construct
GGLGSDTLI

SEQ ID NO: 6062 - protein, 9 aa, synthetic construct
GGYGNDVVS

SEQ ID NO: 6063 - protein, 9 aa, synthetic construct
GGSGHDKLL

SEQ ID NO: 6064 - protein, 9 aa, synthetic construct
GGAGHDLLL

SEQ ID NO: 6065 - protein, 9 aa, synthetic construct
GGAGADEFV

SEQ ID NO: 6066 - protein, 9 aa, synthetic construct
GGNGDDSLT

SEQ ID NO: 6067 - protein, 9 aa, synthetic construct
GGLGSDTYV

SEQ ID NO: 6068 - protein, 9 aa, synthetic construct
GGNGNDVVS

SEQ ID NO: 6069 - protein, 9 aa, synthetic construct
GGAGNDIVR

SEQ ID NO: 6070 - protein, 9 aa, synthetic construct
GGNGNDVVT

SEQ ID NO: 6071 - protein, 9 aa, synthetic construct
GGTGDDLLE

SEQ ID NO: 6072 - protein, 9 aa, synthetic construct
GGAGNDIFD

SEQ ID NO: 6073 - protein, 9 aa, synthetic construct
GGAGNDLYY

SEQ ID NO: 6074 - protein, 9 aa, synthetic construct
GGNGNDTLG

SEQ ID NO: 6075 - protein, 9 aa, synthetic construct
GGAGNDHLV

SEQ ID NO: 6076 - protein, 9 aa, synthetic construct
GGSGGDYIN

SEQ ID NO: 6077 - protein, 9 aa, synthetic construct
GGEGNDIID

SEQ ID NO: 6078 - protein, 9 aa, synthetic construct
GGAGHDILI

SEQ ID NO: 6079 - protein, 9 aa, synthetic construct
GGEGNDHLF

SEQ ID NO: 6080 - protein, 9 aa, synthetic construct
GGAGADFLV

SEQ ID NO: 6081 - protein, 9 aa, synthetic construct
GGTGDDLLW

SEQ ID NO: 6082 - protein, 9 aa, synthetic construct
GGDGNDQLL

SEQ ID NO: 6083 - protein, 9 aa, synthetic construct
GGNGRDILR

SEQ ID NO: 6084 - protein, 9 aa, synthetic construct
GGDGNDQLN

SEQ ID NO: 6085 - protein, 9 aa, synthetic construct
GGAGNDLVR

SEQ ID NO: 6086 - protein, 9 aa, synthetic construct
GGGGSDRFV

SEQ ID NO: 6087 - protein, 9 aa, synthetic construct
GGLGSDTIF

SEQ ID NO: 6088 - protein, 9 aa, synthetic construct
GGAGHDLLE

SEQ ID NO: 6089 - protein, 9 aa, synthetic construct
GGYGSDTYI

SEQ ID NO: 6090 - protein, 9 aa, synthetic construct
GGAGHDLIQ

SEQ ID NO: 6091 - protein, 9 aa, synthetic construct
GGTGADTYL

SEQ ID NO: 6092 - protein, 9 aa, synthetic construct
GGAGKDTVN

SEQ ID NO: 6093 - protein, 9 aa, synthetic construct
GGTGADVLI

SEQ ID NO: 6094 - protein, 9 aa, synthetic construct
GGGGGDILV

SEQ ID NO: 6095 - protein, 9 aa, synthetic construct
GGKGNDRLT

SEQ ID NO: 6096 - protein, 9 aa, synthetic construct
GGNGDDALI

SEQ ID NO: 6097 - protein, 9 aa, synthetic construct
GGAGADALA

SEQ ID NO: 6098 - protein, 9 aa, synthetic construct
GGAGKDVLW

SEQ ID NO: 6099 - protein, 9 aa, synthetic construct
GGGGSDTLH

SEQ ID NO: 6100 - protein, 9 aa, synthetic construct
GGTGDDTYT

SEQ ID NO: 6101 - protein, 9 aa, synthetic construct
GGTGDDTYR

SEQ ID NO: 6102 - protein, 9 aa, synthetic construct
GGNGQDVLY

SEQ ID NO: 6103 - protein, 9 aa, synthetic construct
GGTGDDTFV

SEQ ID NO: 6104 - protein, 9 aa, synthetic construct
GGYGVDTVI

SEQ ID NO: 6105 - protein, 9 aa, synthetic construct
GGAGHDVLS

SEQ ID NO: 6106 - protein, 9 aa, synthetic construct
GGTGADVFL

SEQ ID NO: 6107 - protein, 9 aa, synthetic construct
GGYGNDTLQ

SEQ ID NO: 6108 - protein, 9 aa, synthetic construct
GGEGKDILV

SEQ ID NO: 6109 - protein, 9 aa, synthetic construct
GGEGADTMT

SEQ ID NO: 6110 - protein, 9 aa, synthetic construct
GGGGSDTIK

SEQ ID NO: 6111 - protein, 9 aa, synthetic construct
GGNGNDVLH

SEQ ID NO: 6112 - protein, 9 aa, synthetic construct
GGNGDDYLE

SEQ ID NO: 6113 - protein, 9 aa, synthetic construct
GGAGADELQ

SEQ ID NO: 6114 - protein, 9 aa, synthetic construct
GGSGDDSMS

SEQ ID NO: 6115 - protein, 9 aa, synthetic construct
GGAGNDNLI

SEQ ID NO: 6116 - protein, 9 aa, synthetic construct
GGLGSDTFQ

SEQ ID NO: 6117 - protein, 9 aa, synthetic construct
GGEGDDWLL

SEQ ID NO: 6118 - protein, 9 aa, synthetic construct
GGKGNDSLD

SEQ ID NO: 6119 - protein, 9 aa, synthetic construct
GGTGDDVLE

SEQ ID NO: 6120 - protein, 9 aa, synthetic construct
GGGGNDVIS

SEQ ID NO: 6121 - protein, 9 aa, synthetic construct
GGNGNDSLH

SEQ ID NO: 6122 - protein, 9 aa, synthetic construct
GGAGHDTLF

SEQ ID NO: 6123 - protein, 9 aa, synthetic construct
GGTGADVMY

SEQ ID NO: 6124 - protein, 9 aa, synthetic construct
GGTGDDDLT

SEQ ID NO: 6125 - protein, 9 aa, synthetic construct
GGAGADELY

SEQ ID NO: 6126 - protein, 9 aa, synthetic construct
GGSGGDTFI

SEQ ID NO: 6127 - protein, 9 aa, synthetic construct
GGTGADVMR

SEQ ID NO: 6128 - protein, 9 aa, synthetic construct
GGKGNDILE

SEQ ID NO: 6129 - protein, 9 aa, synthetic construct
GGLGNDTVT

SEQ ID NO: 6130 - protein, 9 aa, synthetic construct
GGNGNDTIV

SEQ ID NO: 6131 - protein, 9 aa, synthetic construct
GGIGRDYLN

SEQ ID NO: 6132 - protein, 9 aa, synthetic construct
GGAGNDKIT

SEQ ID NO: 6133 - protein, 9 aa, synthetic construct
GGTGADSLN

SEQ ID NO: 6134 - protein, 9 aa, synthetic construct
GGDGDDQLI

SEQ ID NO: 6135 - protein, 9 aa, synthetic construct
GGNGNDTMT

SEQ ID NO: 6136 - protein, 9 aa, synthetic construct
GGTGADVLS

SEQ ID NO: 6137 - protein, 9 aa, synthetic construct
GGTGDDSYV

SEQ ID NO: 6138 - protein, 9 aa, synthetic construct
GGLGSDTLL

SEQ ID NO: 6139 - protein, 9 aa, synthetic construct
GGTGDDVVN

SEQ ID NO: 6140 - protein, 9 aa, synthetic construct
GGTGNDVFR

SEQ ID NO: 6141 - protein, 9 aa, synthetic construct
GGAGKDVLK

SEQ ID NO: 6142 - protein, 9 aa, synthetic construct
GGSGNDSIE

SEQ ID NO: 6143 - protein, 9 aa, synthetic construct
GGSGNDIIT

SEQ ID NO: 6144 - protein, 9 aa, synthetic construct
GGNGHDVLS

SEQ ID NO: 6145 - protein, 9 aa, synthetic construct
GGRGDDQLS

SEQ ID NO: 6146 - protein, 9 aa, synthetic construct
GGAGDDWIA

SEQ ID NO: 6147 - protein, 9 aa, synthetic construct
GGGGNDILH

SEQ ID NO: 6148 - protein, 9 aa, synthetic construct
GGFGNDLLS

SEQ ID NO: 6149 - protein, 9 aa, synthetic construct
GGAGRDQLW

SEQ ID NO: 6150 - protein, 9 aa, synthetic construct
GGLGNDALR

SEQ ID NO: 6151 - protein, 9 aa, synthetic construct
GGAGDDVVV

SEQ ID NO: 6152 - protein, 9 aa, synthetic construct
GGPGHDTLL

SEQ ID NO: 6153 - protein, 9 aa, synthetic construct
GGDGSDTIL

SEQ ID NO: 6154 - protein, 9 aa, synthetic construct
GGAGDDVVL

SEQ ID NO: 6155 - protein, 9 aa, synthetic construct
GGAGDDVVK

SEQ ID NO: 6156 - protein, 9 aa, synthetic construct
GGRGDDLLA

SEQ ID NO: 6157 - protein, 9 aa, synthetic construct
GGGGDDQLF

SEQ ID NO: 6158 - protein, 9 aa, synthetic construct
GGAGDDVMS

SEQ ID NO: 6159 - protein, 9 aa, synthetic construct
GGRGDDILI

SEQ ID NO: 6160 - protein, 9 aa, synthetic construct
GGIGADTLV

SEQ ID NO: 6161 - protein, 9 aa, synthetic construct
GGDGDDLIR

SEQ ID NO: 6162 - protein, 9 aa, synthetic construct
GGSGRDAFV

SEQ ID NO: 6163 - protein, 9 aa, synthetic construct
GGKGGDTLA

SEQ ID NO: 6164 - protein, 9 aa, synthetic construct
GGAGIDTAI

SEQ ID NO: 6165 - protein, 9 aa, synthetic construct
GGPGSDYLV

SEQ ID NO: 6166 - protein, 9 aa, synthetic construct
GGDGSDSLT

SEQ ID NO: 6167 - protein, 9 aa, synthetic construct
GGTGRDTLV

SEQ ID NO: 6168 - protein, 9 aa, synthetic construct
GGDGHDVLI

SEQ ID NO: 6169 - protein, 9 aa, synthetic construct
GGDGGDTLD

SEQ ID NO: 6170 - protein, 9 aa, synthetic construct
GGAGDDKLW

SEQ ID NO: 6171 - protein, 9 aa, synthetic construct
GGSGNDTVN

SEQ ID NO: 6172 - protein, 9 aa, synthetic construct
GGAGRDLLR

SEQ ID NO: 6173 - protein, 9 aa, synthetic construct
GGSGNDHLS

SEQ ID NO: 6174 - protein, 9 aa, synthetic construct
GGDGVDTLD

SEQ ID NO: 6175 - protein, 9 aa, synthetic construct
GGDGDDLIL

SEQ ID NO: 6176 - protein, 9 aa, synthetic construct
GGLGSDLLT

SEQ ID NO: 6177 - protein, 9 aa, synthetic construct
GGRGDDSLL

SEQ ID NO: 6178 - protein, 9 aa, synthetic construct
GGAGDDWLS

SEQ ID NO: 6179 - protein, 9 aa, synthetic construct
GGVGNDVIS

SEQ ID NO: 6180 - protein, 9 aa, synthetic construct
GGSGNDIIL

SEQ ID NO: 6181 - protein, 9 aa, synthetic construct
GGRGDDILD

SEQ ID NO: 6182 - protein, 9 aa, synthetic construct
GGLGNDALN

SEQ ID NO: 6183 - protein, 9 aa, synthetic construct
GGTGSDRID

SEQ ID NO: 6184 - protein, 9 aa, synthetic construct
GGAGRDRLN

SEQ ID NO: 6185 - protein, 9 aa, synthetic construct
GGAGDDVIQ

SEQ ID NO: 6186 - protein, 9 aa, synthetic construct
GGGGRDVLT

SEQ ID NO: 6187 - protein, 9 aa, synthetic construct
GGVGNDVLT

SEQ ID NO: 6188 - protein, 9 aa, synthetic construct
GGEGRDTLA

SEQ ID NO: 6189 - protein, 9 aa, synthetic construct
GGDGDDELS

SEQ ID NO: 6190 - protein, 9 aa, synthetic construct
GGAGVDRLT

SEQ ID NO: 6191 - protein, 9 aa, synthetic construct
GGAGSDSID

SEQ ID NO: 6192 - protein, 9 aa, synthetic construct
GGAGDDVFI

SEQ ID NO: 6193 - protein, 9 aa, synthetic construct
GGVGVDVLS

SEQ ID NO: 6194 - protein, 9 aa, synthetic construct
GGFGDDVLN

SEQ ID NO: 6195 - protein, 9 aa, synthetic construct
GGAGVDRLE

SEQ ID NO: 6196 - protein, 9 aa, synthetic construct
GGAGVDRLD

SEQ ID NO: 6197 - protein, 9 aa, synthetic construct
GGRGADTLS

SEQ ID NO: 6198 - protein, 9 aa, synthetic construct
GGRGADTLL

SEQ ID NO: 6199 - protein, 9 aa, synthetic construct
GGAGSDSFV

SEQ ID NO: 6200 - protein, 9 aa, synthetic construct
GGAGTDTAI

SEQ ID NO: 6201 - protein, 9 aa, synthetic construct
GGGGADQLS

SEQ ID NO: 6202 - protein, 9 aa, synthetic construct
GGPGKDTLI

SEQ ID NO: 6203 - protein, 9 aa, synthetic construct
GGAGADTVL

SEQ ID NO: 6204 - protein, 9 aa, synthetic construct
GGVGDDVLY

SEQ ID NO: 6205 - protein, 9 aa, synthetic construct
GGAGADTVA

SEQ ID NO: 6206 - protein, 9 aa, synthetic construct
GGDGSDTIY

SEQ ID NO: 6207 - protein, 9 aa, synthetic construct
GGSGSDRMS

SEQ ID NO: 6208 - protein, 9 aa, synthetic construct
GGGGDDQIF

SEQ ID NO: 6209 - protein, 9 aa, synthetic construct
GGFGHDLLD

SEQ ID NO: 6210 - protein, 9 aa, synthetic construct
GGSGNDVVQ

SEQ ID NO: 6211 - protein, 9 aa, synthetic construct
GGLGDDEIF

SEQ ID NO: 6212 - protein, 9 aa, synthetic construct
GGAGIDTLE

SEQ ID NO: 6213 - protein, 9 aa, synthetic construct
GGAGADTVD

SEQ ID NO: 6214 - protein, 9 aa, synthetic construct
GGTGSDTID

SEQ ID NO: 6215 - protein, 9 aa, synthetic construct
GGGGNDIIN

SEQ ID NO: 6216 - protein, 9 aa, synthetic construct
GGAGSDSLI

SEQ ID NO: 6217 - protein, 9 aa, synthetic construct
GGAGVDSLI

SEQ ID NO: 6218 - protein, 9 aa, synthetic construct
GGSGSDLLD

SEQ ID NO: 6219 - protein, 9 aa, synthetic construct
GGDGDDLIT

SEQ ID NO: 6220 - protein, 9 aa, synthetic construct
GGGGIDTLV

SEQ ID NO: 6221 - protein, 9 aa, synthetic construct
GGVGDDVYV

SEQ ID NO: 6222 - protein, 9 aa, synthetic construct
GGTGRDTFV

SEQ ID NO: 6223 - protein, 9 aa, synthetic construct
GGLGADVIR

SEQ ID NO: 6224 - protein, 9 aa, synthetic construct
GGLGLDTLT

SEQ ID NO: 6225 - protein, 9 aa, synthetic construct
GGTGNDYLF

SEQ ID NO: 6226 - protein, 9 aa, synthetic construct
GGTGNDYME

SEQ ID NO: 6227 - protein, 9 aa, synthetic construct
GGGGDDRLI

SEQ ID NO: 6228 - protein, 9 aa, synthetic construct
GGAGSDTVS

SEQ ID NO: 6229 - protein, 9 aa, synthetic construct
GGSGNDSLK

SEQ ID NO: 6230 - protein, 9 aa, synthetic construct
GGRGNDKLI

SEQ ID NO: 6231 - protein, 9 aa, synthetic construct
GGAGEDSLN

SEQ ID NO: 6232 - protein, 9 aa, synthetic construct
GGAGEDSLL

SEQ ID NO: 6233 - protein, 9 aa, synthetic construct
GGAGQDTLL

SEQ ID NO: 6234 - protein, 9 aa, synthetic construct
GGEGRDSLY

SEQ ID NO: 6235 - protein, 9 aa, synthetic construct
GGDGADYLD

SEQ ID NO: 6236 - protein, 9 aa, synthetic construct
GGRGNDILV

SEQ ID NO: 6237 - protein, 9 aa, synthetic construct
GGAGADSFI

SEQ ID NO: 6238 - protein, 9 aa, synthetic construct
GGAGSDTMY

SEQ ID NO: 6239 - protein, 9 aa, synthetic construct
GGAGQDTLW

SEQ ID NO: 6240 - protein, 9 aa, synthetic construct
GGDGDDLIF

SEQ ID NO: 6241 - protein, 9 aa, synthetic construct
GGKGDDTYL

SEQ ID NO: 6242 - protein, 9 aa, synthetic construct
GGDGSDNLF

SEQ ID NO: 6243 - protein, 9 aa, synthetic construct
GGTGNDYLV

SEQ ID NO: 6244 - protein, 9 aa, synthetic construct
GGAGNDAIY

SEQ ID NO: 6245 - protein, 9 aa, synthetic construct
GGTGRDSLF

SEQ ID NO: 6246 - protein, 9 aa, synthetic construct
GGDGNDFLN

SEQ ID NO: 6247 - protein, 9 aa, synthetic construct
GGPGDDTVR

SEQ ID NO: 6248 - protein, 9 aa, synthetic construct
GGGGDDRLW

SEQ ID NO: 6249 - protein, 9 aa, synthetic construct
GGLGADLLT

SEQ ID NO: 6250 - protein, 9 aa, synthetic construct
GGVGDDKLY

SEQ ID NO: 6251 - protein, 9 aa, synthetic construct
GGTGNDVVT

SEQ ID NO: 6252 - protein, 9 aa, synthetic construct
GGSGNDDLY

SEQ ID NO: 6253 - protein, 9 aa, synthetic construct
GGRGNDQLY

SEQ ID NO: 6254 - protein, 9 aa, synthetic construct
GGAGKDRLF

SEQ ID NO: 6255 - protein, 9 aa, synthetic construct
GGSGSDIFV

SEQ ID NO: 6256 - protein, 9 aa, synthetic construct
GGRGNDNLF

SEQ ID NO: 6257 - protein, 9 aa, synthetic construct
GGTGNDWLS

SEQ ID NO: 6258 - protein, 9 aa, synthetic construct
GGAGQDTAV

SEQ ID NO: 6259 - protein, 9 aa, synthetic construct
GGRGNDLYQ

SEQ ID NO: 6260 - protein, 9 aa, synthetic construct
GGSGNDSLQ

SEQ ID NO: 6261 - protein, 9 aa, synthetic construct
GGAGEDTFK

SEQ ID NO: 6262 - protein, 9 aa, synthetic construct
GGDGNDFLQ

SEQ ID NO: 6263 - protein, 9 aa, synthetic construct
GGTGNDYIE

SEQ ID NO: 6264 - protein, 9 aa, synthetic construct
GGAGSDTML

SEQ ID NO: 6265 - protein, 9 aa, synthetic construct
GGFGNDTIN

SEQ ID NO: 6266 - protein, 9 aa, synthetic construct
GGFGNDTIL

SEQ ID NO: 6267 - protein, 9 aa, synthetic construct
GGRGMDILR

SEQ ID NO: 6268 - protein, 9 aa, synthetic construct
GGDGVDTLY

SEQ ID NO: 6269 - protein, 9 aa, synthetic construct
GGDGSDRLF

SEQ ID NO: 6270 - protein, 9 aa, synthetic construct
GGAGRDILN

SEQ ID NO: 6271 - protein, 9 aa, synthetic construct
GGGGDDQLY

SEQ ID NO: 6272 - protein, 9 aa, synthetic construct
GGEGDDALF

SEQ ID NO: 6273 - protein, 9 aa, synthetic construct
GGLGDDYLE

SEQ ID NO: 6274 - protein, 9 aa, synthetic construct
GGAGSDTIV

SEQ ID NO: 6275 - protein, 9 aa, synthetic construct
GGAGRDKLK

SEQ ID NO: 6276 - protein, 9 aa, synthetic construct
GGGGADVVI

SEQ ID NO: 6277 - protein, 9 aa, synthetic construct
GGDGNDTAV

SEQ ID NO: 6278 - protein, 9 aa, synthetic construct
GGSGNDGLR

SEQ ID NO: 6279 - protein, 9 aa, synthetic construct
GGAGRDKLV

SEQ ID NO: 6280 - protein, 9 aa, synthetic construct
GGEGDDALQ

SEQ ID NO: 6281 - protein, 9 aa, synthetic construct
GGEGDDALS

SEQ ID NO: 6282 - protein, 9 aa, synthetic construct
GGDGNDTFF

SEQ ID NO: 6283 - protein, 9 aa, synthetic construct
GGAGEDALF

SEQ ID NO: 6284 - protein, 9 aa, synthetic construct
GGSGSDYLS

SEQ ID NO: 6285 - protein, 9 aa, synthetic construct
GGNGNDLLS

SEQ ID NO: 6286 - protein, 9 aa, synthetic construct
GGAGEDIFV

SEQ ID NO: 6287 - protein, 9 aa, synthetic construct
GGGGLDTLD

SEQ ID NO: 6288 - protein, 9 aa, synthetic construct
GGEGDDVIN

SEQ ID NO: 6289 - protein, 9 aa, synthetic construct
GGAGDDDLV

SEQ ID NO: 6290 - protein, 9 aa, synthetic construct
GGFGDDTYY

SEQ ID NO: 6291 - protein, 9 aa, synthetic construct
GGLGADRMA

SEQ ID NO: 6292 - protein, 9 aa, synthetic construct
GGKGHDLLI

SEQ ID NO: 6293 - protein, 9 aa, synthetic construct
GGTGQDTLS

SEQ ID NO: 6294 - protein, 9 aa, synthetic construct
GGKGHDLLD

SEQ ID NO: 6295 - protein, 9 aa, synthetic construct
GGDGDDFLD

SEQ ID NO: 6296 - protein, 9 aa, synthetic construct
GGDGNDELS

SEQ ID NO: 6297 - protein, 9 aa, synthetic construct
GGDGNDEIV

SEQ ID NO: 6298 - protein, 9 aa, synthetic construct
GGLGADSLL

SEQ ID NO: 6299 - protein, 9 aa, synthetic construct
GGSGNDFLS

SEQ ID NO: 6300 - protein, 9 aa, synthetic construct
GGIGDDKLF

SEQ ID NO: 6301 - protein, 9 aa, synthetic construct
GGSGNDFLY

SEQ ID NO: 6302 - protein, 9 aa, synthetic construct
GGGGADKLE

SEQ ID NO: 6303 - protein, 9 aa, synthetic construct
GGNGNDLLW

SEQ ID NO: 6304 - protein, 9 aa, synthetic construct
GGAGRDFLT

SEQ ID NO: 6305 - protein, 9 aa, synthetic construct
GGLGDDVLL

SEQ ID NO: 6306 - protein, 9 aa, synthetic construct
GGAGDDDIS

SEQ ID NO: 6307 - protein, 9 aa, synthetic construct
GGAGLDTLY

SEQ ID NO: 6308 - protein, 9 aa, synthetic construct
GGAGSDILK

SEQ ID NO: 6309 - protein, 9 aa, synthetic construct
GGAGTDTLL

SEQ ID NO: 6310 - protein, 9 aa, synthetic construct
GGDGLDTLY

SEQ ID NO: 6311 - protein, 9 aa, synthetic construct
GGDGDDDLL

SEQ ID NO: 6312 - protein, 9 aa, synthetic construct
GGDGDDYIS

SEQ ID NO: 6313 - protein, 9 aa, synthetic construct
GGKGDDVLN

SEQ ID NO: 6314 - protein, 9 aa, synthetic construct
GGVGNDYMD

SEQ ID NO: 6315 - protein, 9 aa, synthetic construct
GGSGTDTAT

SEQ ID NO: 6316 - protein, 9 aa, synthetic construct
GGVGRDVLT

SEQ ID NO: 6317 - protein, 9 aa, synthetic construct
GGVGADSLA

SEQ ID NO: 6318 - protein, 9 aa, synthetic construct
GGVGDDRMD

SEQ ID NO: 6319 - protein, 9 aa, synthetic construct
GGSGSDRLF

SEQ ID NO: 6320 - protein, 9 aa, synthetic construct
GGQGNDTVY

SEQ ID NO: 6321 - protein, 9 aa, synthetic construct
GGKGDDVLV

SEQ ID NO: 6322 - protein, 9 aa, synthetic construct
GGDGIDTLS

SEQ ID NO: 6323 - protein, 9 aa, synthetic construct
GGSGTDSLY

SEQ ID NO: 6324 - protein, 9 aa, synthetic construct
GGDGTDALS

SEQ ID NO: 6325 - protein, 9 aa, synthetic construct
GGGGRDIIY

SEQ ID NO: 6326 - protein, 9 aa, synthetic construct
GGAGDDQLV

SEQ ID NO: 6327 - protein, 9 aa, synthetic construct
GGHGADTLI

SEQ ID NO: 6328 - protein, 9 aa, synthetic construct
GGPGNDTYV

SEQ ID NO: 6329 - protein, 9 aa, synthetic construct
GGSGSDRLL

SEQ ID NO: 6330 - protein, 9 aa, synthetic construct
GGPGNDVIS

SEQ ID NO: 6331 - protein, 9 aa, synthetic construct
GGAGTDTID

SEQ ID NO: 6332 - protein, 9 aa, synthetic construct
GGSGTDTVT

SEQ ID NO: 6333 - protein, 9 aa, synthetic construct
GGSGNDVIA

SEQ ID NO: 6334 - protein, 9 aa, synthetic construct
GGPGNDVLI

SEQ ID NO: 6335 - protein, 9 aa, synthetic construct
GGPGNDVLM

SEQ ID NO: 6336 - protein, 9 aa, synthetic construct
GGAGDDLLG

SEQ ID NO: 6337 - protein, 9 aa, synthetic construct
GGEGRDVLE

SEQ ID NO: 6338 - protein, 9 aa, synthetic construct
GGLGDDQLT

SEQ ID NO: 6339 - protein, 9 aa, synthetic construct
GGQGQDYLY

SEQ ID NO: 6340 - protein, 9 aa, synthetic construct
GGGGDDLIE

SEQ ID NO: 6341 - protein, 9 aa, synthetic construct
GGVGDDSLL

SEQ ID NO: 6342 - protein, 9 aa, synthetic construct
GGDGDDDLR

SEQ ID NO: 6343 - protein, 9 aa, synthetic construct
GGDGSDYLD

SEQ ID NO: 6344 - protein, 9 aa, synthetic construct
GGAGSDIFF

SEQ ID NO: 6345 - protein, 9 aa, synthetic construct
GGAGDDLLM

SEQ ID NO: 6346 - protein, 9 aa, synthetic construct
GGSGNDNLD

SEQ ID NO: 6347 - protein, 9 aa, synthetic construct
GGVGDDRLF

SEQ ID NO: 6348 - protein, 9 aa, synthetic construct
GGQGNDTLQ

SEQ ID NO: 6349 - protein, 9 aa, synthetic construct
GGAGTDYLS

SEQ ID NO: 6350 - protein, 9 aa, synthetic construct
GGLGIDQLT

SEQ ID NO: 6351 - protein, 9 aa, synthetic construct
GGAGDDNLF

SEQ ID NO: 6352 - protein, 9 aa, synthetic construct
GGAGKDEIL

SEQ ID NO: 6353 - protein, 9 aa, synthetic construct
GGEGSDSIS

SEQ ID NO: 6354 - protein, 9 aa, synthetic construct
GGEGDDVII

SEQ ID NO: 6355 - protein, 9 aa, synthetic construct
GGQGNDRLF

SEQ ID NO: 6356 - protein, 9 aa, synthetic construct
GGFGNDNLI

SEQ ID NO: 6357 - protein, 9 aa, synthetic construct
GGAGSDLLQ

SEQ ID NO: 6358 - protein, 9 aa, synthetic construct
GGEGRDWLY

SEQ ID NO: 6359 - protein, 9 aa, synthetic construct
GGGGDDILL

SEQ ID NO: 6360 - protein, 9 aa, synthetic construct
GGVGDDLLI

SEQ ID NO: 6361 - protein, 9 aa, synthetic construct
GGAGDDAIY

SEQ ID NO: 6362 - protein, 9 aa, synthetic construct
GGDGNDTMY

SEQ ID NO: 6363 - protein, 9 aa, synthetic construct
GGAGDDMLR

SEQ ID NO: 6364 - protein, 9 aa, synthetic construct
GGLGDDTIS

SEQ ID NO: 6365 - protein, 9 aa, synthetic construct
GGGGNDFIR

SEQ ID NO: 6366 - protein, 9 aa, synthetic construct
GGSGNDRII

SEQ ID NO: 6367 - protein, 9 aa, synthetic construct
GGFGNDMLS

SEQ ID NO: 6368 - protein, 9 aa, synthetic construct
GGAGDDLYL

SEQ ID NO: 6369 - protein, 9 aa, synthetic construct
GGSGNDRLQ

SEQ ID NO: 6370 - protein, 9 aa, synthetic construct
GGGGDDILS

SEQ ID NO: 6371 - protein, 9 aa, synthetic construct
GGNGKDRLV

SEQ ID NO: 6372 - protein, 9 aa, synthetic construct
GGEGNDALN

SEQ ID NO: 6373 - protein, 9 aa, synthetic construct
GGDGDDYIN

SEQ ID NO: 6374 - protein, 9 aa, synthetic construct
GGVGADTLY

SEQ ID NO: 6375 - protein, 9 aa, synthetic construct
GGPGRDFLT

SEQ ID NO: 6376 - protein, 9 aa, synthetic construct
GGDGDDYIL

SEQ ID NO: 6377 - protein, 9 aa, synthetic construct
GGEGSDSLV

SEQ ID NO: 6378 - protein, 9 aa, synthetic construct
GGVGDDQIY

SEQ ID NO: 6379 - protein, 9 aa, synthetic construct
GGPGRDIFV

SEQ ID NO: 6380 - protein, 9 aa, synthetic construct
GGVGDDLYV

SEQ ID NO: 6381 - protein, 9 aa, synthetic construct
GGAGDDLVQ

SEQ ID NO: 6382 - protein, 9 aa, synthetic construct
GGEGSDSLL

SEQ ID NO: 6383 - protein, 9 aa, synthetic construct
GGDGIDTLL

SEQ ID NO: 6384 - protein, 9 aa, synthetic construct
GGGGRDIVL

SEQ ID NO: 6385 - protein, 9 aa, synthetic construct
GGAGSDLIE

SEQ ID NO: 6386 - protein, 9 aa, synthetic construct
GGSGTDRVD

SEQ ID NO: 6387 - protein, 9 aa, synthetic construct
GGMGKDTLT

SEQ ID NO: 6388 - protein, 9 aa, synthetic construct
GGNGNDILS

SEQ ID NO: 6389 - protein, 9 aa, synthetic construct
GGQGLDSLF

SEQ ID NO: 6390 - protein, 9 aa, synthetic construct
GGQGKDLLS

SEQ ID NO: 6391 - protein, 9 aa, synthetic construct
GGRGADLID

SEQ ID NO: 6392 - protein, 9 aa, synthetic construct
GGDGIDHIK

SEQ ID NO: 6393 - protein, 9 aa, synthetic construct
GGAGDDTIQ

SEQ ID NO: 6394 - protein, 9 aa, synthetic construct
GGDGIDILV

SEQ ID NO: 6395 - protein, 9 aa, synthetic construct
GGEGADVLD

SEQ ID NO: 6396 - protein, 9 aa, synthetic construct
GGEGADLLA

SEQ ID NO: 6397 - protein, 9 aa, synthetic construct
GGLGDDVIR

SEQ ID NO: 6398 - protein, 9 aa, synthetic construct
GGTGTDTLT

SEQ ID NO: 6399 - protein, 9 aa, synthetic construct
GGRGADDFV

SEQ ID NO: 6400 - protein, 9 aa, synthetic construct
GGDGNDTVN

SEQ ID NO: 6401 - protein, 9 aa, synthetic construct
GGPGNDMLI

SEQ ID NO: 6402 - protein, 9 aa, synthetic construct
GGLGDDKLF

SEQ ID NO: 6403 - protein, 9 aa, synthetic construct
GGQGVDVIY

SEQ ID NO: 6404 - protein, 9 aa, synthetic construct
GGDGIDLLD

SEQ ID NO: 6405 - protein, 9 aa, synthetic construct
GGAGRDVVS

SEQ ID NO: 6406 - protein, 9 aa, synthetic construct
GGDGDDEIH

SEQ ID NO: 6407 - protein, 9 aa, synthetic construct
GGAGIDWAD

SEQ ID NO: 6408 - protein, 9 aa, synthetic construct
GGAGRDWVR

SEQ ID NO: 6409 - protein, 9 aa, synthetic construct
GGAGDDTLG

SEQ ID NO: 6410 - protein, 9 aa, synthetic construct
GGVGDDTYI

SEQ ID NO: 6411 - protein, 9 aa, synthetic construct
GGAGDDLIQ

SEQ ID NO: 6412 - protein, 9 aa, synthetic construct
GGDGSDTVY

SEQ ID NO: 6413 - protein, 9 aa, synthetic construct
GGDGDDELI

SEQ ID NO: 6414 - protein, 9 aa, synthetic construct
GGAGADVFK

SEQ ID NO: 6415 - protein, 9 aa, synthetic construct
GGAGVDRFV

SEQ ID NO: 6416 - protein, 9 aa, synthetic construct
GGLGLDTLS

SEQ ID NO: 6417 - protein, 9 aa, synthetic construct
GGSGNDRVY

SEQ ID NO: 6418 - protein, 9 aa, synthetic construct
GGAGTDTAR

SEQ ID NO: 6419 - protein, 9 aa, synthetic construct
GGAGDDTVY

SEQ ID NO: 6420 - protein, 9 aa, synthetic construct
GGAGDDTVV

SEQ ID NO: 6421 - protein, 9 aa, synthetic construct
GGAGVDQLY

SEQ ID NO: 6422 - protein, 9 aa, synthetic construct
GGRGADRLY

SEQ ID NO: 6423 - protein, 9 aa, synthetic construct
GGDGNDTIQ

SEQ ID NO: 6424 - protein, 9 aa, synthetic construct
GGLGDDVLA

SEQ ID NO: 6425 - protein, 9 aa, synthetic construct
GGVGDDTYL

SEQ ID NO: 6426 - protein, 9 aa, synthetic construct
GGAGADVIH

SEQ ID NO: 6427 - protein, 9 aa, synthetic construct
GGAGADVIL

SEQ ID NO: 6428 - protein, 9 aa, synthetic construct
GGSGNDLII

SEQ ID NO: 6429 - protein, 9 aa, synthetic construct
GGAGADVIR

SEQ ID NO: 6430 - protein, 9 aa, synthetic construct
GGEGSDTLY

SEQ ID NO: 6431 - protein, 9 aa, synthetic construct
GGGGDDLLT

SEQ ID NO: 6432 - protein, 9 aa, synthetic construct
GGNGDDLLE

SEQ ID NO: 6433 - protein, 9 aa, synthetic construct
GGMGNDVYI

SEQ ID NO: 6434 - protein, 9 aa, synthetic construct
GGEGSDTIY

SEQ ID NO: 6435 - protein, 9 aa, synthetic construct
GGGGADSFA

SEQ ID NO: 6436 - protein, 9 aa, synthetic construct
GGEGDDVIF

SEQ ID NO: 6437 - protein, 9 aa, synthetic construct
GGEGNDEIY

SEQ ID NO: 6438 - protein, 9 aa, synthetic construct
GGGGNDSLA

SEQ ID NO: 6439 - protein, 9 aa, synthetic construct
GGLGDDLMV

SEQ ID NO: 6440 - protein, 9 aa, synthetic construct
GGFGNDRLT

SEQ ID NO: 6441 - protein, 9 aa, synthetic construct
GGLGDDLYI

SEQ ID NO: 6442 - protein, 9 aa, synthetic construct
GGLGDDLYV

SEQ ID NO: 6443 - protein, 9 aa, synthetic construct
GGVGDDTLE

SEQ ID NO: 6444 - protein, 9 aa, synthetic construct
GGNGNDGLT

SEQ ID NO: 6445 - protein, 9 aa, synthetic construct
GGAGADWLE

SEQ ID NO: 6446 - protein, 9 aa, synthetic construct
GGAGSDRLI

SEQ ID NO: 6447 - protein, 9 aa, synthetic construct
GGDGSDVYV

SEQ ID NO: 6448 - protein, 9 aa, synthetic construct
GGGGADSIV

SEQ ID NO: 6449 - protein, 9 aa, synthetic construct
GGLGDDMYV

SEQ ID NO: 6450 - protein, 9 aa, synthetic construct
GGDGNDYLI

SEQ ID NO: 6451 - protein, 9 aa, synthetic construct
GGDGSDVLR

SEQ ID NO: 6452 - protein, 9 aa, synthetic construct
GGAGSDDLD

SEQ ID NO: 6453 - protein, 9 aa, synthetic construct
GGLGDDLML

SEQ ID NO: 6454 - protein, 9 aa, synthetic construct
GGAGVDKLS

SEQ ID NO: 6455 - protein, 9 aa, synthetic construct
GGEGRDTLT

SEQ ID NO: 6456 - protein, 9 aa, synthetic construct
GGAGRDYLT

SEQ ID NO: 6457 - protein, 9 aa, synthetic construct
GGTGVDLIY

SEQ ID NO: 6458 - protein, 9 aa, synthetic construct
GGPGNDRLE

SEQ ID NO: 6459 - protein, 9 aa, synthetic construct
GGAGDDSLW

SEQ ID NO: 6460 - protein, 9 aa, synthetic construct
GGPGNDRLL

SEQ ID NO: 6461 - protein, 9 aa, synthetic construct
GGVGSDVLL

SEQ ID NO: 6462 - protein, 9 aa, synthetic construct
GGAGSDRLV

SEQ ID NO: 6463 - protein, 9 aa, synthetic construct
GGDGMDLLA

SEQ ID NO: 6464 - protein, 9 aa, synthetic construct
GGLGDDLLE

SEQ ID NO: 6465 - protein, 9 aa, synthetic construct
GGPGNDRMT

SEQ ID NO: 6466 - protein, 9 aa, synthetic construct
GGVGSDTLV

SEQ ID NO: 6467 - protein, 9 aa, synthetic construct
GGDGIDTVV

SEQ ID NO: 6468 - protein, 9 aa, synthetic construct
GGTGVDTFD

SEQ ID NO: 6469 - protein, 9 aa, synthetic construct
GGAGDDSII

SEQ ID NO: 6470 - protein, 9 aa, synthetic construct
GGKGFDWAV

SEQ ID NO: 6471 - protein, 9 aa, synthetic construct
GGAGWDTLD

SEQ ID NO: 6472 - protein, 9 aa, synthetic construct
GGRGNDRLR

SEQ ID NO: 6473 - protein, 9 aa, synthetic construct
GGLGADLLI

SEQ ID NO: 6474 - protein, 9 aa, synthetic construct
GGGGDDVMT

SEQ ID NO: 6475 - protein, 9 aa, synthetic construct
GGAGADLFT

SEQ ID NO: 6476 - protein, 9 aa, synthetic construct
GGSGNDTFT

SEQ ID NO: 6477 - protein, 9 aa, synthetic construct
GGAGSDYLG

SEQ ID NO: 6478 - protein, 9 aa, synthetic construct
GGSGRDVLT

SEQ ID NO: 6479 - protein, 9 aa, synthetic construct
GGQGDDLID

SEQ ID NO: 6480 - protein, 9 aa, synthetic construct
GGDGADVFI

SEQ ID NO: 6481 - protein, 9 aa, synthetic construct
GGYGDDLFI

SEQ ID NO: 6482 - protein, 9 aa, synthetic construct
GGGGDDVLF

SEQ ID NO: 6483 - protein, 9 aa, synthetic construct
GGQGDDLLF

SEQ ID NO: 6484 - protein, 9 aa, synthetic construct
GGIGNDALN

SEQ ID NO: 6485 - protein, 9 aa, synthetic construct
GGSGADSLI

SEQ ID NO: 6486 - protein, 9 aa, synthetic construct
GGSGADSIS

SEQ ID NO: 6487 - protein, 9 aa, synthetic construct
GGDGRDTVY

SEQ ID NO: 6488 - protein, 9 aa, synthetic construct
GGQGDDLLT

SEQ ID NO: 6489 - protein, 9 aa, synthetic construct
GGGGNDYLH

SEQ ID NO: 6490 - protein, 9 aa, synthetic construct
GGDGNDLLK

SEQ ID NO: 6491 - protein, 9 aa, synthetic construct
GGNGADTLA

SEQ ID NO: 6492 - protein, 9 aa, synthetic construct
GGVGNDFLD

SEQ ID NO: 6493 - protein, 9 aa, synthetic construct
GGEGRDLFV

SEQ ID NO: 6494 - protein, 9 aa, synthetic construct
GGVGNDILF

SEQ ID NO: 6495 - protein, 9 aa, synthetic construct
GGEGDDFLS

SEQ ID NO: 6496 - protein, 9 aa, synthetic construct
GGEGNDLLT

SEQ ID NO: 6497 - protein, 9 aa, synthetic construct
GGGGRDRLD

SEQ ID NO: 6498 - protein, 9 aa, synthetic construct
GGEGNDLLV

SEQ ID NO: 6499 - protein, 9 aa, synthetic construct
GGEGADTIY

SEQ ID NO: 6500 - protein, 9 aa, synthetic construct
GGAGADKFL

SEQ ID NO: 6501 - protein, 9 aa, synthetic construct
GGEGADILR

SEQ ID NO: 6502 - protein, 9 aa, synthetic construct
GGSGNDTIG

SEQ ID NO: 6503 - protein, 9 aa, synthetic construct
GGDGADILT

SEQ ID NO: 6504 - protein, 9 aa, synthetic construct
GGDGRDTID

SEQ ID NO: 6505 - protein, 9 aa, synthetic construct
GGGGDDWLD

SEQ ID NO: 6506 - protein, 9 aa, synthetic construct
GGDGEDTLL

SEQ ID NO: 6507 - protein, 9 aa, synthetic construct
GGYGDDTID

SEQ ID NO: 6508 - protein, 9 aa, synthetic construct
GGTGIDTLD

SEQ ID NO: 6509 - protein, 9 aa, synthetic construct
GGDGDDILK

SEQ ID NO: 6510 - protein, 9 aa, synthetic construct
GGEGDDYLS

SEQ ID NO: 6511 - protein, 9 aa, synthetic construct
GGNGADTLY

SEQ ID NO: 6512 - protein, 9 aa, synthetic construct
GGGGGDTLD

SEQ ID NO: 6513 - protein, 9 aa, synthetic construct
GGAGNDTVA

SEQ ID NO: 6514 - protein, 9 aa, synthetic construct
GGLGNDQLN

SEQ ID NO: 6515 - protein, 9 aa, synthetic construct
GGSGKDTLT

SEQ ID NO: 6516 - protein, 9 aa, synthetic construct
GGNGYDIYI

SEQ ID NO: 6517 - protein, 9 aa, synthetic construct
GGDGADDIG

SEQ ID NO: 6518 - protein, 9 aa, synthetic construct
GGIGIDTMY

SEQ ID NO: 6519 - protein, 9 aa, synthetic construct
GGDGNDLIL

SEQ ID NO: 6520 - protein, 9 aa, synthetic construct
GGEGDDVIT

SEQ ID NO: 6521 - protein, 9 aa, synthetic construct
GGSGKDVLY

SEQ ID NO: 6522 - protein, 9 aa, synthetic construct
GGSGADLLI

SEQ ID NO: 6523 - protein, 9 aa, synthetic construct
GGTGADIFY

SEQ ID NO: 6524 - protein, 9 aa, synthetic construct
GGTGLDTLT

SEQ ID NO: 6525 - protein, 9 aa, synthetic construct
GGDGDDSIG

SEQ ID NO: 6526 - protein, 9 aa, synthetic construct
GGDGKDVFI

SEQ ID NO: 6527 - protein, 9 aa, synthetic construct
GGQGDDRLD

SEQ ID NO: 6528 - protein, 9 aa, synthetic construct
GGPGADLLD

SEQ ID NO: 6529 - protein, 9 aa, synthetic construct
GGDGSDAVR

SEQ ID NO: 6530 - protein, 9 aa, synthetic construct
GGAGFDTLI

SEQ ID NO: 6531 - protein, 9 aa, synthetic construct
GGAGEDTLS

SEQ ID NO: 6532 - protein, 9 aa, synthetic construct
GGGGPDQMA

SEQ ID NO: 6533 - protein, 9 aa, synthetic construct
GGAGLDKLY

SEQ ID NO: 6534 - protein, 9 aa, synthetic construct
GGDGKDTLS

SEQ ID NO: 6535 - protein, 9 aa, synthetic construct
GGSGADMLF

SEQ ID NO: 6536 - protein, 9 aa, synthetic construct
GGDGNDLIT

SEQ ID NO: 6537 - protein, 9 aa, synthetic construct
GGAGNDTYA

SEQ ID NO: 6538 - protein, 9 aa, synthetic construct
GGQGADIMA

SEQ ID NO: 6539 - protein, 9 aa, synthetic construct
GGSGADRLE

SEQ ID NO: 6540 - protein, 9 aa, synthetic construct
GGTGADIMI

SEQ ID NO: 6541 - protein, 9 aa, synthetic construct
GGEGSDILA

SEQ ID NO: 6542 - protein, 9 aa, synthetic construct
GGDGRDVLT

SEQ ID NO: 6543 - protein, 9 aa, synthetic construct
GGTGKDVFV

SEQ ID NO: 6544 - protein, 9 aa, synthetic construct
GGGGHDTLR

SEQ ID NO: 6545 - protein, 9 aa, synthetic construct
GGDGKDTLD

SEQ ID NO: 6546 - protein, 9 aa, synthetic construct
GGDGADDLS

SEQ ID NO: 6547 - protein, 9 aa, synthetic construct
GGLGHDEIY

SEQ ID NO: 6548 - protein, 9 aa, synthetic construct
GGAGDDGLF

SEQ ID NO: 6549 - protein, 9 aa, synthetic construct
GGAGFDYAS

SEQ ID NO: 6550 - protein, 9 aa, synthetic construct
GGAGNDTYN

SEQ ID NO: 6551 - protein, 9 aa, synthetic construct
GGAGADLMS

SEQ ID NO: 6552 - protein, 9 aa, synthetic construct
GGEGDDLIF

SEQ ID NO: 6553 - protein, 9 aa, synthetic construct
GGAGNDTYW

SEQ ID NO: 6554 - protein, 9 aa, synthetic construct
GGAGGDMLD

SEQ ID NO: 6555 - protein, 9 aa, synthetic construct
GGIGNDILR

SEQ ID NO: 6556 - protein, 9 aa, synthetic construct
GGGGDDTYV

SEQ ID NO: 6557 - protein, 9 aa, synthetic construct
GGSGDDNLY

SEQ ID NO: 6558 - protein, 9 aa, synthetic construct
GGYGNDELN

SEQ ID NO: 6559 - protein, 9 aa, synthetic construct
GGAGNDRLM

SEQ ID NO: 6560 - protein, 9 aa, synthetic construct
GGSGSDTLA

SEQ ID NO: 6561 - protein, 9 aa, synthetic construct
GGSGDDMLS

SEQ ID NO: 6562 - protein, 9 aa, synthetic construct
GGAGADHLV

SEQ ID NO: 6563 - protein, 9 aa, synthetic construct
GGVGNDLLN

SEQ ID NO: 6564 - protein, 9 aa, synthetic construct
GGKGDDNLL

SEQ ID NO: 6565 - protein, 9 aa, synthetic construct
GGSGDDLLE

SEQ ID NO: 6566 - protein, 9 aa, synthetic construct
GGAGDDFIA

SEQ ID NO: 6567 - protein, 9 aa, synthetic construct
GGLGNDTIH

SEQ ID NO: 6568 - protein, 9 aa, synthetic construct
GGKGKDTFV

SEQ ID NO: 6569 - protein, 9 aa, synthetic construct
GGSGDDLFR

SEQ ID NO: 6570 - protein, 9 aa, synthetic construct
GGAGDDELQ

SEQ ID NO: 6571 - protein, 9 aa, synthetic construct
GGLGNDTIE

SEQ ID NO: 6572 - protein, 9 aa, synthetic construct
GGSGKDAFV

SEQ ID NO: 6573 - protein, 9 aa, synthetic construct
GGSGSDTID

SEQ ID NO: 6574 - protein, 9 aa, synthetic construct
GGTGGDLLS

SEQ ID NO: 6575 - protein, 9 aa, synthetic construct
GGYGNDELY

SEQ ID NO: 6576 - protein, 9 aa, synthetic construct
GGIGSDTLI

SEQ ID NO: 6577 - protein, 9 aa, synthetic construct
GGGGDDYID

SEQ ID NO: 6578 - protein, 9 aa, synthetic construct
GGAGNDRIV

SEQ ID NO: 6579 - protein, 9 aa, synthetic construct
GGGGSDKFV

SEQ ID NO: 6580 - protein, 9 aa, synthetic construct
GGGGNDVLK

SEQ ID NO: 6581 - protein, 9 aa, synthetic construct
GGEGKDKIS

SEQ ID NO: 6582 - protein, 9 aa, synthetic construct
GGAGNDRFI

SEQ ID NO: 6583 - protein, 9 aa, synthetic construct
GGGGDDFIF

SEQ ID NO: 6584 - protein, 9 aa, synthetic construct
GGDGNDYVD

SEQ ID NO: 6585 - protein, 9 aa, synthetic construct
GGVGNDMLF

SEQ ID NO: 6586 - protein, 9 aa, synthetic construct
GGEGADIFV

SEQ ID NO: 6587 - protein, 9 aa, synthetic construct
GGNGRDTLS

SEQ ID NO: 6588 - protein, 9 aa, synthetic construct
GGAGDDELV

SEQ ID NO: 6589 - protein, 9 aa, synthetic construct
GGAGADGYA

SEQ ID NO: 6590 - protein, 9 aa, synthetic construct
GGGGHDTLY

SEQ ID NO: 6591 - protein, 9 aa, synthetic construct
GGQGADTVE

SEQ ID NO: 6592 - protein, 9 aa, synthetic construct
GGSGDDQLT

SEQ ID NO: 6593 - protein, 9 aa, synthetic construct
GGGGSDVIW

SEQ ID NO: 6594 - protein, 9 aa, synthetic construct
GGFGADSIS

SEQ ID NO: 6595 - protein, 9 aa, synthetic construct
GGSGDDQFS

SEQ ID NO: 6596 - protein, 9 aa, synthetic construct
GGSGSDTFT

SEQ ID NO: 6597 - protein, 9 aa, synthetic construct
GGFGSDTFV

SEQ ID NO: 6598 - protein, 9 aa, synthetic construct
GGSGDDIMV

SEQ ID NO: 6599 - protein, 9 aa, synthetic construct
GGAGGDTIT

SEQ ID NO: 6600 - protein, 9 aa, synthetic construct
GGDGKDRLF

SEQ ID NO: 6601 - protein, 9 aa, synthetic construct
GGNGSDTFI

SEQ ID NO: 6602 - protein, 9 aa, synthetic construct
GGAGDDELA

SEQ ID NO: 6603 - protein, 9 aa, synthetic construct
GGTGADLLT

SEQ ID NO: 6604 - protein, 9 aa, synthetic construct
GGYGEDTLK

SEQ ID NO: 6605 - protein, 9 aa, synthetic construct
GGEGADVLS

SEQ ID NO: 6606 - protein, 9 aa, synthetic construct
GGAGNDSVL

SEQ ID NO: 6607 - protein, 9 aa, synthetic construct
GGAGNDSVN

SEQ ID NO: 6608 - protein, 9 aa, synthetic construct
GGSGDDAVG

SEQ ID NO: 6609 - protein, 9 aa, synthetic construct
GGTGADLLL

SEQ ID NO: 6610 - protein, 9 aa, synthetic construct
GGSGSDTLR

SEQ ID NO: 6611 - protein, 9 aa, synthetic construct
GGNGDDVIY

SEQ ID NO: 6612 - protein, 9 aa, synthetic construct
GGTGHDTLR

SEQ ID NO: 6613 - protein, 9 aa, synthetic construct
GGNGNDRLV

SEQ ID NO: 6614 - protein, 9 aa, synthetic construct
GGNGNDALN

SEQ ID NO: 6615 - protein, 9 aa, synthetic construct
GGLGNDSLE

SEQ ID NO: 6616 - protein, 9 aa, synthetic construct
GGAGDDFLL

SEQ ID NO: 6617 - protein, 9 aa, synthetic construct
GGDGRDSLF

SEQ ID NO: 6618 - protein, 9 aa, synthetic construct
GGSGDDELT

SEQ ID NO: 6619 - protein, 9 aa, synthetic construct
GGNGSDSLL

SEQ ID NO: 6620 - protein, 9 aa, synthetic construct
GGAGADIIN

SEQ ID NO: 6621 - protein, 9 aa, synthetic construct
GGFGSDTLI

SEQ ID NO: 6622 - protein, 9 aa, synthetic construct
GGTGGDTLD

SEQ ID NO: 6623 - protein, 9 aa, synthetic construct
GGQGDDALA

SEQ ID NO: 6624 - protein, 9 aa, synthetic construct
GGGGDDDLY

SEQ ID NO: 6625 - protein, 9 aa, synthetic construct
GGTGGDTLV

SEQ ID NO: 6626 - protein, 9 aa, synthetic construct
GGSGRDTLT

SEQ ID NO: 6627 - protein, 9 aa, synthetic construct
GGAGDDFIY

SEQ ID NO: 6628 - protein, 9 aa, synthetic construct
GGDGADLLY

SEQ ID NO: 6629 - protein, 9 aa, synthetic construct
GGYGFDVLL

SEQ ID NO: 6630 - protein, 9 aa, synthetic construct
GGQGDDELD

SEQ ID NO: 6631 - protein, 9 aa, synthetic construct
GGAGGDSLS

SEQ ID NO: 6632 - protein, 9 aa, synthetic construct
GGVGNDILT

SEQ ID NO: 6633 - protein, 9 aa, synthetic construct
GGDGADLLS

SEQ ID NO: 6634 - protein, 9 aa, synthetic construct
GGIGNDLLT

SEQ ID NO: 6635 - protein, 9 aa, synthetic construct
GGDGHDLIE

SEQ ID NO: 6636 - protein, 9 aa, synthetic construct
GGTGHDILD

SEQ ID NO: 6637 - protein, 9 aa, synthetic construct
GGDGDDIIV

SEQ ID NO: 6638 - protein, 9 aa, synthetic construct
GGDGDDIIW

SEQ ID NO: 6639 - protein, 9 aa, synthetic construct
GGLGNDMVS

SEQ ID NO: 6640 - protein, 9 aa, synthetic construct
GGKGHDTLV

SEQ ID NO: 6641 - protein, 9 aa, synthetic construct
GGAGKDLFK

SEQ ID NO: 6642 - protein, 9 aa, synthetic construct
GGLGXDYLQ

SEQ ID NO: 6643 - protein, 9 aa, synthetic construct
GGIGDDVLN

SEQ ID NO: 6644 - protein, 9 aa, synthetic construct
GGLGRDVLD

SEQ ID NO: 6645 - protein, 9 aa, synthetic construct
GGTGNDQVS

SEQ ID NO: 6646 - protein, 9 aa, synthetic construct
GGIGDDVLI

SEQ ID NO: 6647 - protein, 9 aa, synthetic construct
GGEGNDRLL

SEQ ID NO: 6648 - protein, 9 aa, synthetic construct
GGFGNDTLL

SEQ ID NO: 6649 - protein, 9 aa, synthetic construct
GGIGDDVLS

SEQ ID NO: 6650 - protein, 9 aa, synthetic construct
GGNGGDTLI

SEQ ID NO: 6651 - protein, 9 aa, synthetic construct
GGSGNDSMV

SEQ ID NO: 6652 - protein, 9 aa, synthetic construct
GGQGDDTYV

SEQ ID NO: 6653 - protein, 9 aa, synthetic construct
GGTGNDRLA

SEQ ID NO: 6654 - protein, 9 aa, synthetic construct
GGGGADDLN

SEQ ID NO: 6655 - protein, 9 aa, synthetic construct
GGGGADDLR

SEQ ID NO: 6656 - protein, 9 aa, synthetic construct
GGGGADDLS

SEQ ID NO: 6657 - protein, 9 aa, synthetic construct
GGNGDDTFV

SEQ ID NO: 6658 - protein, 9 aa, synthetic construct
GGFGNDTLR

SEQ ID NO: 6659 - protein, 9 aa, synthetic construct
GGAGSDVIN

SEQ ID NO: 6660 - protein, 9 aa, synthetic construct
GGAGNDDLA

SEQ ID NO: 6661 - protein, 9 aa, synthetic construct
GGEGDDTVI

SEQ ID NO: 6662 - protein, 9 aa, synthetic construct
GGPGDDIMT

SEQ ID NO: 6663 - protein, 9 aa, synthetic construct
GGEGNDVLF

SEQ ID NO: 6664 - protein, 9 aa, synthetic construct
GGGGHDVLD

SEQ ID NO: 6665 - protein, 9 aa, synthetic construct
GGTGNDMLY

SEQ ID NO: 6666 - protein, 9 aa, synthetic construct
GGTGADEFV

SEQ ID NO: 6667 - protein, 9 aa, synthetic construct
GGEGVDGLR

SEQ ID NO: 6668 - protein, 9 aa, synthetic construct
GGQGDDTLA

SEQ ID NO: 6669 - protein, 9 aa, synthetic construct
GGPGDDLLE

SEQ ID NO: 6670 - protein, 9 aa, synthetic construct
GGEGDDTVS

SEQ ID NO: 6671 - protein, 9 aa, synthetic construct
GGRGRDVLL

SEQ ID NO: 6672 - protein, 9 aa, synthetic construct
GGKGYDHLT

SEQ ID NO: 6673 - protein, 9 aa, synthetic construct
GGEGCDIFQ

SEQ ID NO: 6674 - protein, 9 aa, synthetic construct
GGAGNDDID

SEQ ID NO: 6675 - protein, 9 aa, synthetic construct
GGEGCDLLD

SEQ ID NO: 6676 - protein, 9 aa, synthetic construct
GGTGNDQLA

SEQ ID NO: 6677 - protein, 9 aa, synthetic construct
GGDGSDLLD

SEQ ID NO: 6678 - protein, 9 aa, synthetic construct
GGAGQDLLL

SEQ ID NO: 6679 - protein, 9 aa, synthetic construct
GGDGNDIIW

SEQ ID NO: 6680 - protein, 9 aa, synthetic construct
GGNGNDFLD

SEQ ID NO: 6681 - protein, 9 aa, synthetic construct
GGLGNDIID

SEQ ID NO: 6682 - protein, 9 aa, synthetic construct
GGDGVDVLL

SEQ ID NO: 6683 - protein, 9 aa, synthetic construct
GGSGSDVLV

SEQ ID NO: 6684 - protein, 9 aa, synthetic construct
GGTGNDTME

SEQ ID NO: 6685 - protein, 9 aa, synthetic construct
GGTGNDTMF

SEQ ID NO: 6686 - protein, 9 aa, synthetic construct
GGIGDDTLY

SEQ ID NO: 6687 - protein, 9 aa, synthetic construct
GGTGNDTMN

SEQ ID NO: 6688 - protein, 9 aa, synthetic construct
GGQGDDVLT

SEQ ID NO: 6689 - protein, 9 aa, synthetic construct
GGGGDDSIT

SEQ ID NO: 6690 - protein, 9 aa, synthetic construct
GGFGDDTLV

SEQ ID NO: 6691 - protein, 9 aa, synthetic construct
GGNGDDTYL

SEQ ID NO: 6692 - protein, 9 aa, synthetic construct
GGDGDDAMF

SEQ ID NO: 6693 - protein, 9 aa, synthetic construct
GGTGNDTYW

SEQ ID NO: 6694 - protein, 9 aa, synthetic construct
GGAGADRLG

SEQ ID NO: 6695 - protein, 9 aa, synthetic construct
GGSGNDTMI

SEQ ID NO: 6696 - protein, 9 aa, synthetic construct
GGRGNDSLS

SEQ ID NO: 6697 - protein, 9 aa, synthetic construct
GGSGNDSLW

SEQ ID NO: 6698 - protein, 9 aa, synthetic construct
GGWGNDSVS

SEQ ID NO: 6699 - protein, 9 aa, synthetic construct
GGAGLDRMT

SEQ ID NO: 6700 - protein, 9 aa, synthetic construct
GGWGNDTLR

SEQ ID NO: 6701 - protein, 9 aa, synthetic construct
GGIGDDVAV

SEQ ID NO: 6702 - protein, 9 aa, synthetic construct
GGTGNDSLA

SEQ ID NO: 6703 - protein, 9 aa, synthetic construct
GGWGNDVID

SEQ ID NO: 6704 - protein, 9 aa, synthetic construct
GGSGSDVLN

SEQ ID NO: 6705 - protein, 9 aa, synthetic construct
GGLGADILR

SEQ ID NO: 6706 - protein, 9 aa, synthetic construct
GGGGDDSLI

SEQ ID NO: 6707 - protein, 9 aa, synthetic construct
GGLGADIMI

SEQ ID NO: 6708 - protein, 9 aa, synthetic construct
GGRGNDVLR

SEQ ID NO: 6709 - protein, 9 aa, synthetic construct
GGTGNDTIK

SEQ ID NO: 6710 - protein, 9 aa, synthetic construct
GGTGNDSVS

SEQ ID NO: 6711 - protein, 9 aa, synthetic construct
GGLGNDILF

SEQ ID NO: 6712 - protein, 9 aa, synthetic construct
GGTGNDSYF

SEQ ID NO: 6713 - protein, 9 aa, synthetic construct
GGAGEDVFV

SEQ ID NO: 6714 - protein, 9 aa, synthetic construct
GGVGIDTLI

SEQ ID NO: 6715 - protein, 9 aa, synthetic construct
GGDGDDALY

SEQ ID NO: 6716 - protein, 9 aa, synthetic construct
GGTGNDTFY

SEQ ID NO: 6717 - protein, 9 aa, synthetic construct
GGDGNDIIQ

SEQ ID NO: 6718 - protein, 9 aa, synthetic construct
GGEGADSLL

SEQ ID NO: 6719 - protein, 9 aa, synthetic construct
GGRGSDQLW

SEQ ID NO: 6720 - protein, 9 aa, synthetic construct
GGEGNDQLW

SEQ ID NO: 6721 - protein, 9 aa, synthetic construct
GGLGTDILI

SEQ ID NO: 6722 - protein, 9 aa, synthetic construct
GGLGNDLLR

SEQ ID NO: 6723 - protein, 9 aa, synthetic construct
GGQGDDSLT

SEQ ID NO: 6724 - protein, 9 aa, synthetic construct
GGDGNDKLN

SEQ ID NO: 6725 - protein, 9 aa, synthetic construct
GGAGNDWIH

SEQ ID NO: 6726 - protein, 9 aa, synthetic construct
GGDGDDSLM

SEQ ID NO: 6727 - protein, 9 aa, synthetic construct
GGDGNDKLA

SEQ ID NO: 6728 - protein, 9 aa, synthetic construct
GGDGHDRLW

SEQ ID NO: 6729 - protein, 9 aa, synthetic construct
GGLGNDLLS

SEQ ID NO: 6730 - protein, 9 aa, synthetic construct
GGNGADRLA

SEQ ID NO: 6731 - protein, 9 aa, synthetic construct
GGTGNDHIE

SEQ ID NO: 6732 - protein, 9 aa, synthetic construct
GGGGDDTLK

SEQ ID NO: 6733 - protein, 9 aa, synthetic construct
GGFGNDTVN

SEQ ID NO: 6734 - protein, 9 aa, synthetic construct
GGAGADNLY

SEQ ID NO: 6735 - protein, 9 aa, synthetic construct
GGEGADKIN

SEQ ID NO: 6736 - protein, 9 aa, synthetic construct
GGDGNDIVN

SEQ ID NO: 6737 - protein, 9 aa, synthetic construct
GGQGDDSID

SEQ ID NO: 6738 - protein, 9 aa, synthetic construct
GGEGNDQLI

SEQ ID NO: 6739 - protein, 9 aa, synthetic construct
GGDGNDVIR

SEQ ID NO: 6740 - protein, 9 aa, synthetic construct
GGAGNDEIN

SEQ ID NO: 6741 - protein, 9 aa, synthetic construct
GGSGSDVFR

SEQ ID NO: 6742 - protein, 9 aa, synthetic construct
GGTGNDALF

SEQ ID NO: 6743 - protein, 9 aa, synthetic construct
GGDGHDRLS

SEQ ID NO: 6744 - protein, 9 aa, synthetic construct
GGPGADTFS

SEQ ID NO: 6745 - protein, 9 aa, synthetic construct
GGVGLDTLV

SEQ ID NO: 6746 - protein, 9 aa, synthetic construct
GGNGADSID

SEQ ID NO: 6747 - protein, 9 aa, synthetic construct
GGDGNDLAS

SEQ ID NO: 6748 - protein, 9 aa, synthetic construct
GGTGNDDLQ

SEQ ID NO: 6749 - protein, 9 aa, synthetic construct
GGNGDDRLT

SEQ ID NO: 6750 - protein, 9 aa, synthetic construct
GGAGNDVVF

SEQ ID NO: 6751 - protein, 9 aa, synthetic construct
GGCGADRLF

SEQ ID NO: 6752 - protein, 9 aa, synthetic construct
GGDGKDVFV

SEQ ID NO: 6753 - protein, 9 aa, synthetic construct
GGAGNDEIH

SEQ ID NO: 6754 - protein, 9 aa, synthetic construct
GGLGNDLMS

SEQ ID NO: 6755 - protein, 9 aa, synthetic construct
GGDGSDFLA

SEQ ID NO: 6756 - protein, 9 aa, synthetic construct
GGVGNDSLT

SEQ ID NO: 6757 - protein, 9 aa, synthetic construct
GGDGNDSLW

SEQ ID NO: 6758 - protein, 9 aa, synthetic construct
GGAGNDWLR

SEQ ID NO: 6759 - protein, 9 aa, synthetic construct
GGAGKDSLS

SEQ ID NO: 6760 - protein, 9 aa, synthetic construct
GGDGKDVLN

SEQ ID NO: 6761 - protein, 9 aa, synthetic construct
GGDGNDIMY

SEQ ID NO: 6762 - protein, 9 aa, synthetic construct
GGGGDDTIE

SEQ ID NO: 6763 - protein, 9 aa, synthetic construct
GGAGDDHIV

SEQ ID NO: 6764 - protein, 9 aa, synthetic construct
GGKGSDWLY

SEQ ID NO: 6765 - protein, 9 aa, synthetic construct
GGNGDDVFV

SEQ ID NO: 6766 - protein, 9 aa, synthetic construct
GGLGQDDLI

SEQ ID NO: 6767 - protein, 9 aa, synthetic construct
GGGGSDALF

SEQ ID NO: 6768 - protein, 9 aa, synthetic construct
GGTGNDLIY

SEQ ID NO: 6769 - protein, 9 aa, synthetic construct
GGEGDDTVD

SEQ ID NO: 6770 - protein, 9 aa, synthetic construct
GGDGSDIYI

SEQ ID NO: 6771 - protein, 9 aa, synthetic construct
GGQGDDTIN

SEQ ID NO: 6772 - protein, 9 aa, synthetic construct
GGLGNDKLD

SEQ ID NO: 6773 - protein, 9 aa, synthetic construct
GGDGHDSLL

SEQ ID NO: 6774 - protein, 9 aa, synthetic construct
GGAGPDQMT

SEQ ID NO: 6775 - protein, 9 aa, synthetic construct
GGEGNDRID

SEQ ID NO: 6776 - protein, 9 aa, synthetic construct
GGEGNDRIF

SEQ ID NO: 6777 - protein, 9 aa, synthetic construct
GGSGLDTLL

SEQ ID NO: 6778 - protein, 9 aa, synthetic construct
GGHGNDVLF

SEQ ID NO: 6779 - protein, 9 aa, synthetic construct
GGDGNDIVF

SEQ ID NO: 6780 - protein, 9 aa, synthetic construct
GGGGHDTLD

SEQ ID NO: 6781 - protein, 9 aa, synthetic construct
GGTGNDILF

SEQ ID NO: 6782 - protein, 9 aa, synthetic construct
GGTGNDILK

SEQ ID NO: 6783 - protein, 9 aa, synthetic construct
GGTGNDILQ

SEQ ID NO: 6784 - protein, 9 aa, synthetic construct
GGLGNDLIS

SEQ ID NO: 6785 - protein, 9 aa, synthetic construct
GGGGNDLLT

SEQ ID NO: 6786 - protein, 9 aa, synthetic construct
GGAGNDYLQ

SEQ ID NO: 6787 - protein, 9 aa, synthetic construct
GGGGDDTIL

SEQ ID NO: 6788 - protein, 9 aa, synthetic construct
GGIGTDTLD

SEQ ID NO: 6789 - protein, 9 aa, synthetic construct
GGKGADRLD

SEQ ID NO: 6790 - protein, 9 aa, synthetic construct
GGKGADTLI

SEQ ID NO: 6791 - protein, 9 aa, synthetic construct
GGSGSDSLT

SEQ ID NO: 6792 - protein, 9 aa, synthetic construct
GGAGLDTMD

SEQ ID NO: 6793 - protein, 9 aa, synthetic construct
GGSGSDVLS

SEQ ID NO: 6794 - protein, 9 aa, synthetic construct
GGDGNDTVI

SEQ ID NO: 6795 - protein, 9 aa, synthetic construct
GGTGADTIE

SEQ ID NO: 6796 - protein, 9 aa, synthetic construct
GGSGNDTMA

SEQ ID NO: 6797 - protein, 9 aa, synthetic construct
GGAGKDVLL

SEQ ID NO: 6798 - protein, 9 aa, synthetic construct
GGAGLDTMS

SEQ ID NO: 6799 - protein, 9 aa, synthetic construct
GGSGNDSVL

SEQ ID NO: 6800 - protein, 9 aa, synthetic construct
GGAGKDKLS

SEQ ID NO: 6801 - protein, 9 aa, synthetic construct
GGAGKDVIV

SEQ ID NO: 6802 - protein, 9 aa, synthetic construct
GGAGKDLFL

SEQ ID NO: 6803 - protein, 9 aa, synthetic construct
GGSGSDVLQ

SEQ ID NO: 6804 - protein, 9 aa, synthetic construct
GGSGSDRLT

SEQ ID NO: 6805 - protein, 9 aa, synthetic construct
GGSGNDSFV

SEQ ID NO: 6806 - protein, 9 aa, synthetic construct
GGSGSDTMI

SEQ ID NO: 6807 - protein, 9 aa, synthetic construct
GGSGNDSMS

SEQ ID NO: 6808 - protein, 9 aa, synthetic construct
GGAGKDVLD

SEQ ID NO: 6809 - protein, 9 aa, synthetic construct
GGNGDDTIR

SEQ ID NO: 6810 - protein, 9 aa, synthetic construct
GGKGDDYLS

SEQ ID NO: 6811 - protein, 9 aa, synthetic construct
GGAGKDIMS

SEQ ID NO: 6812 - protein, 9 aa, synthetic construct
GGAGKDKLY

SEQ ID NO: 6813 - protein, 9 aa, synthetic construct
GGSGRDTAS

SEQ ID NO: 6814 - protein, 9 aa, synthetic construct
GGAGKDLLI

SEQ ID NO: 6815 - protein, 9 aa, synthetic construct
GGSGQDRLY

SEQ ID NO: 6816 - protein, 9 aa, synthetic construct
GGFGNDIFQ

SEQ ID NO: 6817 - protein, 9 aa, synthetic construct
GGTGADELI

SEQ ID NO: 6818 - protein, 9 aa, synthetic construct
GGAGKDVAS

SEQ ID NO: 6819 - protein, 9 aa, synthetic construct
GGTGADGMT

SEQ ID NO: 6820 - protein, 9 aa, synthetic construct
GGKGKDAFV

SEQ ID NO: 6821 - protein, 9 aa, synthetic construct
GGGGNDTIG

SEQ ID NO: 6822 - protein, 9 aa, synthetic construct
GGAGNDEIA

SEQ ID NO: 6823 - protein, 9 aa, synthetic construct
GGTGADHLI

SEQ ID NO: 6824 - protein, 9 aa, synthetic construct
GGAGNDEIR

SEQ ID NO: 6825 - protein, 9 aa, synthetic construct
GGDGNDVIV

SEQ ID NO: 6826 - protein, 9 aa, synthetic construct
GGAGNDELE

SEQ ID NO: 6827 - protein, 9 aa, synthetic construct
GGAGKDTVS

SEQ ID NO: 6828 - protein, 9 aa, synthetic construct
GGKGDDSIQ

SEQ ID NO: 6829 - protein, 9 aa, synthetic construct
GGSGKDVLT

SEQ ID NO: 6830 - protein, 9 aa, synthetic construct
GGSGKDVLK

SEQ ID NO: 6831 - protein, 9 aa, synthetic construct
GGAGLDIVS

SEQ ID NO: 6832 - protein, 9 aa, synthetic construct
GGSGRDYID

SEQ ID NO: 6833 - protein, 9 aa, synthetic construct
GGAGNDDLF

SEQ ID NO: 6834 - protein, 9 aa, synthetic construct
GGAGNDDLE

SEQ ID NO: 6835 - protein, 9 aa, synthetic construct
GGAGNDDIQ

SEQ ID NO: 6836 - protein, 9 aa, synthetic construct
GGAGNDHLT

SEQ ID NO: 6837 - protein, 9 aa, synthetic construct
GGAGKDRLL

SEQ ID NO: 6838 - protein, 9 aa, synthetic construct
GGKGHDTFI

SEQ ID NO: 6839 - protein, 9 aa, synthetic construct
GGAGNDHLW

SEQ ID NO: 6840 - protein, 9 aa, synthetic construct
GGSGNDYLN

SEQ ID NO: 6841 - protein, 9 aa, synthetic construct
GGGGNDTFI

SEQ ID NO: 6842 - protein, 9 aa, synthetic construct
GGNGDDRLE

SEQ ID NO: 6843 - protein, 9 aa, synthetic construct
GGAGLDRVL

SEQ ID NO: 6844 - protein, 9 aa, synthetic construct
GGSGNDALH

SEQ ID NO: 6845 - protein, 9 aa, synthetic construct
GGFGNDTLQ

SEQ ID NO: 6846 - protein, 9 aa, synthetic construct
GGTGADALN

SEQ ID NO: 6847 - protein, 9 aa, synthetic construct
GGKGHDTLI

SEQ ID NO: 6848 - protein, 9 aa, synthetic construct
GGSGNDAFH

SEQ ID NO: 6849 - protein, 9 aa, synthetic construct
GGTGADRMY

SEQ ID NO: 6850 - protein, 9 aa, synthetic construct
GGNGDDTYY

SEQ ID NO: 6851 - protein, 9 aa, synthetic construct
GGAGNDAYT

SEQ ID NO: 6852 - protein, 9 aa, synthetic construct
GGKGHDTLN

SEQ ID NO: 6853 - protein, 9 aa, synthetic construct
GGKGDDILN

SEQ ID NO: 6854 - protein, 9 aa, synthetic construct
GGTGADIMD

SEQ ID NO: 6855 - protein, 9 aa, synthetic construct
GGSGNDRIF

SEQ ID NO: 6856 - protein, 9 aa, synthetic construct
GGAGNDHIY

SEQ ID NO: 6857 - protein, 9 aa, synthetic construct
GGSGKDILF

SEQ ID NO: 6858 - protein, 9 aa, synthetic construct
GGSGKDILD

SEQ ID NO: 6859 - protein, 9 aa, synthetic construct
GGAGNDFIV

SEQ ID NO: 6860 - protein, 9 aa, synthetic construct
GGSGKDALR

SEQ ID NO: 6861 - protein, 9 aa, synthetic construct
GGSGKDAID

SEQ ID NO: 6862 - protein, 9 aa, synthetic construct
GGKGDDILH

SEQ ID NO: 6863 - protein, 9 aa, synthetic construct
GGFGNDVMN

SEQ ID NO: 6864 - protein, 9 aa, synthetic construct
GGTGADNMA

SEQ ID NO: 6865 - protein, 9 aa, synthetic construct
GGDGNDVYY

SEQ ID NO: 6866 - protein, 9 aa, synthetic construct
GGAGKDTLQ

SEQ ID NO: 6867 - protein, 9 aa, synthetic construct
GGAGNDGLY

SEQ ID NO: 6868 - protein, 9 aa, synthetic construct
GGDGNDRMV

SEQ ID NO: 6869 - protein, 9 aa, synthetic construct
GGNGDDVMN

SEQ ID NO: 6870 - protein, 9 aa, synthetic construct
GGIGSDTIQ

SEQ ID NO: 6871 - protein, 9 aa, synthetic construct
GGSGIDRMT

SEQ ID NO: 6872 - protein, 9 aa, synthetic construct
GGAGNDGLD

SEQ ID NO: 6873 - protein, 9 aa, synthetic construct
GGTGADQLY

SEQ ID NO: 6874 - protein, 9 aa, synthetic construct
GGLGSDTFA

SEQ ID NO: 6875 - protein, 9 aa, synthetic construct
GGAGNDHID

SEQ ID NO: 6876 - protein, 9 aa, synthetic construct
GGAGNDFIN

SEQ ID NO: 6877 - protein, 9 aa, synthetic construct
GGTGADKIY

SEQ ID NO: 6878 - protein, 9 aa, synthetic construct
GGTGADIVD

SEQ ID NO: 6879 - protein, 9 aa, synthetic construct
GGDGNDSIQ

SEQ ID NO: 6880 - protein, 9 aa, synthetic construct
GGSGRDVLY

SEQ ID NO: 6881 - protein, 9 aa, synthetic construct
GGTGADKFD

SEQ ID NO: 6882 - protein, 9 aa, synthetic construct
GGGGNDTIQ

SEQ ID NO: 6883 - protein, 9 aa, synthetic construct
GGTGADRLN

SEQ ID NO: 6884 - protein, 9 aa, synthetic construct
GGTGADKFV

SEQ ID NO: 6885 - protein, 9 aa, synthetic construct
GGTGADKLD

SEQ ID NO: 6886 - protein, 9 aa, synthetic construct
GGTGADRLA

SEQ ID NO: 6887 - protein, 9 aa, synthetic construct
GGDGNDVLK

SEQ ID NO: 6888 - protein, 9 aa, synthetic construct
GGTGADKMT

SEQ ID NO: 6889 - protein, 9 aa, synthetic construct
GGKGKDLLD

SEQ ID NO: 6890 - protein, 9 aa, synthetic construct
GGTGADLFV

SEQ ID NO: 6891 - protein, 9 aa, synthetic construct
GGTGADLID

SEQ ID NO: 6892 - protein, 9 aa, synthetic construct
GGTGADLIY

SEQ ID NO: 6893 - protein, 9 aa, synthetic construct
GGNGDDVLA

SEQ ID NO: 6894 - protein, 9 aa, synthetic construct
GGSGNDDID

SEQ ID NO: 6895 - protein, 9 aa, synthetic construct
GGAGIDRLL

SEQ ID NO: 6896 - protein, 9 aa, synthetic construct
GGDGQDTLE

SEQ ID NO: 6897 - protein, 9 aa, synthetic construct
GGSGRDRLY

SEQ ID NO: 6898 - protein, 9 aa, synthetic construct
GGKGDDVLL

SEQ ID NO: 6899 - protein, 9 aa, synthetic construct
GGSGHDTLS

SEQ ID NO: 6900 - protein, 9 aa, synthetic construct
GGSGTDTVV

SEQ ID NO: 6901 - protein, 9 aa, synthetic construct
GGEGDDTIV

SEQ ID NO: 6902 - protein, 9 aa, synthetic construct
GGSGNDVIH

SEQ ID NO: 6903 - protein, 9 aa, synthetic construct
GGSGNDVIN

SEQ ID NO: 6904 - protein, 9 aa, synthetic construct
GGNGDDLLS

SEQ ID NO: 6905 - protein, 9 aa, synthetic construct
GGSGNDVIQ

SEQ ID NO: 6906 - protein, 9 aa, synthetic construct
GGNGDDLLR

SEQ ID NO: 6907 - protein, 9 aa, synthetic construct
GGSGNDLMY

SEQ ID NO: 6908 - protein, 9 aa, synthetic construct
GGKGADVFV

SEQ ID NO: 6909 - protein, 9 aa, synthetic construct
GGNGDDLLF

SEQ ID NO: 6910 - protein, 9 aa, synthetic construct
GGAGIDVMD

SEQ ID NO: 6911 - protein, 9 aa, synthetic construct
GGNGDDSLF

SEQ ID NO: 6912 - protein, 9 aa, synthetic construct
GGSGNDLLH

SEQ ID NO: 6913 - protein, 9 aa, synthetic construct
GGSGNDLIL

SEQ ID NO: 6914 - protein, 9 aa, synthetic construct
GGEGNDELT

SEQ ID NO: 6915 - protein, 9 aa, synthetic construct
GGAGLDTLD

SEQ ID NO: 6916 - protein, 9 aa, synthetic construct
GGSGTDTLR

SEQ ID NO: 6917 - protein, 9 aa, synthetic construct
GGKGFDILS

SEQ ID NO: 6918 - protein, 9 aa, synthetic construct
GGSGNDVFD

SEQ ID NO: 6919 - protein, 9 aa, synthetic construct
GGDGNDTMT

SEQ ID NO: 6920 - protein, 9 aa, synthetic construct
GGAGKDLLL

SEQ ID NO: 6921 - protein, 9 aa, synthetic construct
GGFGNDMVD

SEQ ID NO: 6922 - protein, 9 aa, synthetic construct
GGDGNDTMI

SEQ ID NO: 6923 - protein, 9 aa, synthetic construct
GGKGDDVLY

SEQ ID NO: 6924 - protein, 9 aa, synthetic construct
GGNGDDTLM

SEQ ID NO: 6925 - protein, 9 aa, synthetic construct
GGKGDDIYF

SEQ ID NO: 6926 - protein, 9 aa, synthetic construct
GGAGKDLLS

SEQ ID NO: 6927 - protein, 9 aa, synthetic construct
GGSGTDTLD

SEQ ID NO: 6928 - protein, 9 aa, synthetic construct
GGSGTDSLS

SEQ ID NO: 6929 - protein, 9 aa, synthetic construct
GGDGNDTMG

SEQ ID NO: 6930 - protein, 9 aa, synthetic construct
GGFGNDNMN

SEQ ID NO: 6931 - protein, 9 aa, synthetic construct
GGDGNDTMF

SEQ ID NO: 6932 - protein, 9 aa, synthetic construct
GGDGNDTMD

SEQ ID NO: 6933 - protein, 9 aa, synthetic construct
GGSGNDQIF

SEQ ID NO: 6934 - protein, 9 aa, synthetic construct
GGSGNDNLT

SEQ ID NO: 6935 - protein, 9 aa, synthetic construct
GGAGIDTYY

SEQ ID NO: 6936 - protein, 9 aa, synthetic construct
GGSGVDNLS

SEQ ID NO: 6937 - protein, 9 aa, synthetic construct
GGSGSDLLY

SEQ ID NO: 6938 - protein, 9 aa, synthetic construct
GGTGADSLF

SEQ ID NO: 6939 - protein, 9 aa, synthetic construct
GGDGNDVFD

SEQ ID NO: 6940 - protein, 9 aa, synthetic construct
GGGGNDRFR

SEQ ID NO: 6941 - protein, 9 aa, synthetic construct
GGSGRDILD

SEQ ID NO: 6942 - protein, 9 aa, synthetic construct
GGDGDDMLY

SEQ ID NO: 6943 - protein, 9 aa, synthetic construct
GGAGLDTAD

SEQ ID NO: 6944 - protein, 9 aa, synthetic construct
GGLGSDSLS

SEQ ID NO: 6945 - protein, 9 aa, synthetic construct
GGDGNDTAL

SEQ ID NO: 6946 - protein, 9 aa, synthetic construct
GGIGWDTIR

SEQ ID NO: 6947 - protein, 9 aa, synthetic construct
GGNGDDQMQ

SEQ ID NO: 6948 - protein, 9 aa, synthetic construct
GGAGNDAFV

SEQ ID NO: 6949 - protein, 9 aa, synthetic construct
GGSGNDELV

SEQ ID NO: 6950 - protein, 9 aa, synthetic construct
GGSGNDELI

SEQ ID NO: 6951 - protein, 9 aa, synthetic construct
GGLGSDTID

SEQ ID NO: 6952 - protein, 9 aa, synthetic construct
GGAGNDAIT

SEQ ID NO: 6953 - protein, 9 aa, synthetic construct
GGSGSDILD

SEQ ID NO: 6954 - protein, 9 aa, synthetic construct
GGIGVDTLA

SEQ ID NO: 6955 - protein, 9 aa, synthetic construct
GGSGSDKLF

SEQ ID NO: 6956 - protein, 9 aa, synthetic construct
GGEGNDELY

SEQ ID NO: 6957 - protein, 9 aa, synthetic construct
GGDGNDTIM

SEQ ID NO: 6958 - protein, 9 aa, synthetic construct
GGSGNDVVD

SEQ ID NO: 6959 - protein, 9 aa, synthetic construct
GGGGGDRFW

SEQ ID NO: 6960 - protein, 9 aa, synthetic construct
GGDGNDRIS

SEQ ID NO: 6961 - protein, 9 aa, synthetic construct
GGSGNDKLH

SEQ ID NO: 6962 - protein, 9 aa, synthetic construct
GGSGSDLLV

SEQ ID NO: 6963 - protein, 9 aa, synthetic construct
GGAGIDTMA

SEQ ID NO: 6964 - protein, 9 aa, synthetic construct
GGDGNDYIV

SEQ ID NO: 6965 - protein, 9 aa, synthetic construct
GGSGNDVMR

SEQ ID NO: 6966 - protein, 9 aa, synthetic construct
GGKGNDDIT

SEQ ID NO: 6967 - protein, 9 aa, synthetic construct
GGDGNDVFA

SEQ ID NO: 6968 - protein, 9 aa, synthetic construct
GGKGNDDIS

SEQ ID NO: 6969 - protein, 9 aa, synthetic construct
GGDGNDVAL

SEQ ID NO: 6970 - protein, 9 aa, synthetic construct
GGFGNDSLN

SEQ ID NO: 6971 - protein, 9 aa, synthetic construct
GGAGIDTLA

SEQ ID NO: 6972 - protein, 9 aa, synthetic construct
GGKGNDAYV

SEQ ID NO: 6973 - protein, 9 aa, synthetic construct
GGSGVDTLV

SEQ ID NO: 6974 - protein, 9 aa, synthetic construct
GGSGNDIIK

SEQ ID NO: 6975 - protein, 9 aa, synthetic construct
GGSGNDWLQ

SEQ ID NO: 6976 - protein, 9 aa, synthetic construct
GGAGEDMLD

SEQ ID NO: 6977 - protein, 9 aa, synthetic construct
GGDGSDVLI

SEQ ID NO: 6978 - protein, 9 aa, synthetic construct
GGRGDDELH

SEQ ID NO: 6979 - protein, 9 aa, synthetic construct
GGRGDDHLW

SEQ ID NO: 6980 - protein, 9 aa, synthetic construct
GGNGNDLIR

SEQ ID NO: 6981 - protein, 9 aa, synthetic construct
GGTGSDRMF

SEQ ID NO: 6982 - protein, 9 aa, synthetic construct
GGDGSDTLH

SEQ ID NO: 6983 - protein, 9 aa, synthetic construct
GGTGSDSLD

SEQ ID NO: 6984 - protein, 9 aa, synthetic construct
GGTGSDSLT

SEQ ID NO: 6985 - protein, 9 aa, synthetic construct
GGAGRDRME

SEQ ID NO: 6986 - protein, 9 aa, synthetic construct
GGNGNDLIN

SEQ ID NO: 6987 - protein, 9 aa, synthetic construct
GGTGSDTAD

SEQ ID NO: 6988 - protein, 9 aa, synthetic construct
GGLGNDALS

SEQ ID NO: 6989 - protein, 9 aa, synthetic construct
GGLGDDELY

SEQ ID NO: 6990 - protein, 9 aa, synthetic construct
GGEGGDTLD

SEQ ID NO: 6991 - protein, 9 aa, synthetic construct
GGAGADTFF

SEQ ID NO: 6992 - protein, 9 aa, synthetic construct
GGRGDDDLS

SEQ ID NO: 6993 - protein, 9 aa, synthetic construct
GGAGRDSIY

SEQ ID NO: 6994 - protein, 9 aa, synthetic construct
GGDGEDALY

SEQ ID NO: 6995 - protein, 9 aa, synthetic construct
GGAGADTLG

SEQ ID NO: 6996 - protein, 9 aa, synthetic construct
GGAGVDTAI

SEQ ID NO: 6997 - protein, 9 aa, synthetic construct
GGTGSDTLE

SEQ ID NO: 6998 - protein, 9 aa, synthetic construct
GGTGSDTLH

SEQ ID NO: 6999 - protein, 9 aa, synthetic construct
GGRGDDALA

SEQ ID NO: 7000 - protein, 9 aa, synthetic construct
GGLGNDAIF

SEQ ID NO: 7001 - protein, 9 aa, synthetic construct
GGLGDDFLN

SEQ ID NO: 7002 - protein, 9 aa, synthetic construct
GGTGSDTVS

SEQ ID NO: 7003 - protein, 9 aa, synthetic construct
GGTGSDQLS

SEQ ID NO: 7004 - protein, 9 aa, synthetic construct
GGAGDDVVF

SEQ ID NO: 7005 - protein, 9 aa, synthetic construct
GGIGADRVS

SEQ ID NO: 7006 - protein, 9 aa, synthetic construct
GGAGDDWLL

SEQ ID NO: 7007 - protein, 9 aa, synthetic construct
GGRGDDTLN

SEQ ID NO: 7008 - protein, 9 aa, synthetic construct
GGNGNDLLR

SEQ ID NO: 7009 - protein, 9 aa, synthetic construct
GGRGDDTIL

SEQ ID NO: 7010 - protein, 9 aa, synthetic construct
GGRGDDTID

SEQ ID NO: 7011 - protein, 9 aa, synthetic construct
GGRGDDTFI

SEQ ID NO: 7012 - protein, 9 aa, synthetic construct
GGGGVDTLY

SEQ ID NO: 7013 - protein, 9 aa, synthetic construct
GGAGVDVLT

SEQ ID NO: 7014 - protein, 9 aa, synthetic construct
GGNGHDTLY

SEQ ID NO: 7015 - protein, 9 aa, synthetic construct
GGDGNDDLS

SEQ ID NO: 7016 - protein, 9 aa, synthetic construct
GGAGDDWLV

SEQ ID NO: 7017 - protein, 9 aa, synthetic construct
GGAGRDMLR

SEQ ID NO: 7018 - protein, 9 aa, synthetic construct
GGDGNDDLK

SEQ ID NO: 7019 - protein, 9 aa, synthetic construct
GGAGADTAS

SEQ ID NO: 7020 - protein, 9 aa, synthetic construct
GGAGVDTYV

SEQ ID NO: 7021 - protein, 9 aa, synthetic construct
GGAGDDWLF

SEQ ID NO: 7022 - protein, 9 aa, synthetic construct
GGAGDDWLA

SEQ ID NO: 7023 - protein, 9 aa, synthetic construct
GGEGSDVFV

SEQ ID NO: 7024 - protein, 9 aa, synthetic construct
GGGGADMLR

SEQ ID NO: 7025 - protein, 9 aa, synthetic construct
GGAGRDQLF

SEQ ID NO: 7026 - protein, 9 aa, synthetic construct
GGGGNDILF

SEQ ID NO: 7027 - protein, 9 aa, synthetic construct
GGLGDDALD

SEQ ID NO: 7028 - protein, 9 aa, synthetic construct
GGNGHDWLE

SEQ ID NO: 7029 - protein, 9 aa, synthetic construct
GGAGDDVYA

SEQ ID NO: 7030 - protein, 9 aa, synthetic construct
GGPGGDTLI

SEQ ID NO: 7031 - protein, 9 aa, synthetic construct
GGDGDDTMF

SEQ ID NO: 7032 - protein, 9 aa, synthetic construct
GGWGADILD

SEQ ID NO: 7033 - protein, 9 aa, synthetic construct
GGDGDDEID

SEQ ID NO: 7034 - protein, 9 aa, synthetic construct
GGTGTDTMA

SEQ ID NO: 7035 - protein, 9 aa, synthetic construct
GGNGNDKLD

SEQ ID NO: 7036 - protein, 9 aa, synthetic construct
GGPGNDILN

SEQ ID NO: 7037 - protein, 9 aa, synthetic construct
GGRGADIFV

SEQ ID NO: 7038 - protein, 9 aa, synthetic construct
GGGGADRFH

SEQ ID NO: 7039 - protein, 9 aa, synthetic construct
GGAGRDVFN

SEQ ID NO: 7040 - protein, 9 aa, synthetic construct
GGGGKDTLT

SEQ ID NO: 7041 - protein, 9 aa, synthetic construct
GGLGTDTMT

SEQ ID NO: 7042 - protein, 9 aa, synthetic construct
GGGGADRFI

SEQ ID NO: 7043 - protein, 9 aa, synthetic construct
GGTGTDTLD

SEQ ID NO: 7044 - protein, 9 aa, synthetic construct
GGLGVDTLS

SEQ ID NO: 7045 - protein, 9 aa, synthetic construct
GGTGTDTLR

SEQ ID NO: 7046 - protein, 9 aa, synthetic construct
GGAGRDVLL

SEQ ID NO: 7047 - protein, 9 aa, synthetic construct
GGPGNDDVF

SEQ ID NO: 7048 - protein, 9 aa, synthetic construct
GGLGDDIYT

SEQ ID NO: 7049 - protein, 9 aa, synthetic construct
GGEGDDIIV

SEQ ID NO: 7050 - protein, 9 aa, synthetic construct
GGGGADRID

SEQ ID NO: 7051 - protein, 9 aa, synthetic construct
GGDGDDYLV

SEQ ID NO: 7052 - protein, 9 aa, synthetic construct
GGAGRDVVF

SEQ ID NO: 7053 - protein, 9 aa, synthetic construct
GGAGVDLLD

SEQ ID NO: 7054 - protein, 9 aa, synthetic construct
GGEGDDIIG

SEQ ID NO: 7055 - protein, 9 aa, synthetic construct
GGAGDDSYT

SEQ ID NO: 7056 - protein, 9 aa, synthetic construct
GGGGADRLA

SEQ ID NO: 7057 - protein, 9 aa, synthetic construct
GGNGIDTLS

SEQ ID NO: 7058 - protein, 9 aa, synthetic construct
GGEGDDDID

SEQ ID NO: 7059 - protein, 9 aa, synthetic construct
GGAGVDQLT

SEQ ID NO: 7060 - protein, 9 aa, synthetic construct
GGPGNDDIG

SEQ ID NO: 7061 - protein, 9 aa, synthetic construct
GGRGADTLV

SEQ ID NO: 7062 - protein, 9 aa, synthetic construct
GGRGADRME

SEQ ID NO: 7063 - protein, 9 aa, synthetic construct
GGRGADTLM

SEQ ID NO: 7064 - protein, 9 aa, synthetic construct
GGAGDDTYT

SEQ ID NO: 7065 - protein, 9 aa, synthetic construct
GGWGADHMV

SEQ ID NO: 7066 - protein, 9 aa, synthetic construct
GGRGADTLD

SEQ ID NO: 7067 - protein, 9 aa, synthetic construct
GGAGDDTYM

SEQ ID NO: 7068 - protein, 9 aa, synthetic construct
GGAGRDTLG

SEQ ID NO: 7069 - protein, 9 aa, synthetic construct
GGAGDDTYD

SEQ ID NO: 7070 - protein, 9 aa, synthetic construct
GGRGADSLA

SEQ ID NO: 7071 - protein, 9 aa, synthetic construct
GGAGADTYR

SEQ ID NO: 7072 - protein, 9 aa, synthetic construct
GGLGTDTLN

SEQ ID NO: 7073 - protein, 9 aa, synthetic construct
GGLGDDHLD

SEQ ID NO: 7074 - protein, 9 aa, synthetic construct
GGDGSDTVD

SEQ ID NO: 7075 - protein, 9 aa, synthetic construct
GGRGADLLS

SEQ ID NO: 7076 - protein, 9 aa, synthetic construct
GGRGADRLT

SEQ ID NO: 7077 - protein, 9 aa, synthetic construct
GGAGVDRLA

SEQ ID NO: 7078 - protein, 9 aa, synthetic construct
GGRGADRLF

SEQ ID NO: 7079 - protein, 9 aa, synthetic construct
GGAGDDTVA

SEQ ID NO: 7080 - protein, 9 aa, synthetic construct
GGEGDDILE

SEQ ID NO: 7081 - protein, 9 aa, synthetic construct
GGDGDDELF

SEQ ID NO: 7082 - protein, 9 aa, synthetic construct
GGDGSDTVL

SEQ ID NO: 7083 - protein, 9 aa, synthetic construct
GGRGADQLW

SEQ ID NO: 7084 - protein, 9 aa, synthetic construct
GGRGADMLY

SEQ ID NO: 7085 - protein, 9 aa, synthetic construct
GGAGDDTMG

SEQ ID NO: 7086 - protein, 9 aa, synthetic construct
GGDGDDEIY

SEQ ID NO: 7087 - protein, 9 aa, synthetic construct
GGAGDDYIN

SEQ ID NO: 7088 - protein, 9 aa, synthetic construct
GGAGDDYIQ

SEQ ID NO: 7089 - protein, 9 aa, synthetic construct
GGNGNDLLT

SEQ ID NO: 7090 - protein, 9 aa, synthetic construct
GGNGADLLQ

SEQ ID NO: 7091 - protein, 9 aa, synthetic construct
GGAGQDRLF

SEQ ID NO: 7092 - protein, 9 aa, synthetic construct
GGNGADLLS

SEQ ID NO: 7093 - protein, 9 aa, synthetic construct
GGPGDDLLI

SEQ ID NO: 7094 - protein, 9 aa, synthetic construct
GGEGDDVAH

SEQ ID NO: 7095 - protein, 9 aa, synthetic construct
GGTGNDVIN

SEQ ID NO: 7096 - protein, 9 aa, synthetic construct
GGTGNDVIT

SEQ ID NO: 7097 - protein, 9 aa, synthetic construct
GGPGDDLLV

SEQ ID NO: 7098 - protein, 9 aa, synthetic construct
GGTGNDVLK

SEQ ID NO: 7099 - protein, 9 aa, synthetic construct
GGEGRDRLY

SEQ ID NO: 7100 - protein, 9 aa, synthetic construct
GGTGNDVMQ

SEQ ID NO: 7101 - protein, 9 aa, synthetic construct
GGAGEDTLL

SEQ ID NO: 7102 - protein, 9 aa, synthetic construct
GGAGEDTLE

SEQ ID NO: 7103 - protein, 9 aa, synthetic construct
GGAGQDRLE

SEQ ID NO: 7104 - protein, 9 aa, synthetic construct
GGWGNDVYY

SEQ ID NO: 7105 - protein, 9 aa, synthetic construct
GGDGNDFLV

SEQ ID NO: 7106 - protein, 9 aa, synthetic construct
GGGGDDSLV

SEQ ID NO: 7107 - protein, 9 aa, synthetic construct
GGGGDDSLT

SEQ ID NO: 7108 - protein, 9 aa, synthetic construct
GGRGNDLYV

SEQ ID NO: 7109 - protein, 9 aa, synthetic construct
GGGGDDSLN

SEQ ID NO: 7110 - protein, 9 aa, synthetic construct
GGTGNDYID

SEQ ID NO: 7111 - protein, 9 aa, synthetic construct
GGGGDDSLL

SEQ ID NO: 7112 - protein, 9 aa, synthetic construct
GGWGNDTIS

SEQ ID NO: 7113 - protein, 9 aa, synthetic construct
GGLGNDILA

SEQ ID NO: 7114 - protein, 9 aa, synthetic construct
GGGGVDRLI

SEQ ID NO: 7115 - protein, 9 aa, synthetic construct
GGIGDDTLN

SEQ ID NO: 7116 - protein, 9 aa, synthetic construct
GGGGNDKLS

SEQ ID NO: 7117 - protein, 9 aa, synthetic construct
GGRGDDVLF

SEQ ID NO: 7118 - protein, 9 aa, synthetic construct
GGRGNDYLD

SEQ ID NO: 7119 - protein, 9 aa, synthetic construct
GGGGDDTIR

SEQ ID NO: 7120 - protein, 9 aa, synthetic construct
GGTGNDRLR

SEQ ID NO: 7121 - protein, 9 aa, synthetic construct
GGLGADELT

SEQ ID NO: 7122 - protein, 9 aa, synthetic construct
GGEGNDYLA

SEQ ID NO: 7123 - protein, 9 aa, synthetic construct
GGDGNDGLY

SEQ ID NO: 7124 - protein, 9 aa, synthetic construct
GGTGNDRMS

SEQ ID NO: 7125 - protein, 9 aa, synthetic construct
GGLGADFLT

SEQ ID NO: 7126 - protein, 9 aa, synthetic construct
GGAGQDLLD

SEQ ID NO: 7127 - protein, 9 aa, synthetic construct
GGGGDDTII

SEQ ID NO: 7128 - protein, 9 aa, synthetic construct
GGAGYDTAS

SEQ ID NO: 7129 - protein, 9 aa, synthetic construct
GGTGNDSIL

SEQ ID NO: 7130 - protein, 9 aa, synthetic construct
GGAGYDRMY

SEQ ID NO: 7131 - protein, 9 aa, synthetic construct
GGDGGDQFV

SEQ ID NO: 7132 - protein, 9 aa, synthetic construct
GGTGNDSLR

SEQ ID NO: 7133 - protein, 9 aa, synthetic construct
GGLGADILL

SEQ ID NO: 7134 - protein, 9 aa, synthetic construct
GGTGNDSYI

SEQ ID NO: 7135 - protein, 9 aa, synthetic construct
GGAGADQIS

SEQ ID NO: 7136 - protein, 9 aa, synthetic construct
GGEGTDTLT

SEQ ID NO: 7137 - protein, 9 aa, synthetic construct
GGTGNDTIA

SEQ ID NO: 7138 - protein, 9 aa, synthetic construct
GGTGNDTMI

SEQ ID NO: 7139 - protein, 9 aa, synthetic construct
GGPGDDILF

SEQ ID NO: 7140 - protein, 9 aa, synthetic construct
GGLGNDIVD

SEQ ID NO: 7141 - protein, 9 aa, synthetic construct
GGDGADVLA

SEQ ID NO: 7142 - protein, 9 aa, synthetic construct
GGGGKDLLS

SEQ ID NO: 7143 - protein, 9 aa, synthetic construct
GGLGTDSLF

SEQ ID NO: 7144 - protein, 9 aa, synthetic construct
GGLGTDSLT

SEQ ID NO: 7145 - protein, 9 aa, synthetic construct
GGEGDDQLR

SEQ ID NO: 7146 - protein, 9 aa, synthetic construct
GGTGRDRID

SEQ ID NO: 7147 - protein, 9 aa, synthetic construct
GGAGADRMD

SEQ ID NO: 7148 - protein, 9 aa, synthetic construct
GGDGADVLQ

SEQ ID NO: 7149 - protein, 9 aa, synthetic construct
GGLGADTIL

SEQ ID NO: 7150 - protein, 9 aa, synthetic construct
GGPGDDVID

SEQ ID NO: 7151 - protein, 9 aa, synthetic construct
GGRGGDTLE

SEQ ID NO: 7152 - protein, 9 aa, synthetic construct
GGAGADRVF

SEQ ID NO: 7153 - protein, 9 aa, synthetic construct
GGAGRDILD

SEQ ID NO: 7154 - protein, 9 aa, synthetic construct
GGLGVDYLS

SEQ ID NO: 7155 - protein, 9 aa, synthetic construct
GGGGADLID

SEQ ID NO: 7156 - protein, 9 aa, synthetic construct
GGDGHDTLR

SEQ ID NO: 7157 - protein, 9 aa, synthetic construct
GGDGHDTLS

SEQ ID NO: 7158 - protein, 9 aa, synthetic construct
GGAGRDKLL

SEQ ID NO: 7159 - protein, 9 aa, synthetic construct
GGEGNDRYA

SEQ ID NO: 7160 - protein, 9 aa, synthetic construct
GGLGADVFE

SEQ ID NO: 7161 - protein, 9 aa, synthetic construct
GGTGRDRLF

SEQ ID NO: 7162 - protein, 9 aa, synthetic construct
GGDGSDSLF

SEQ ID NO: 7163 - protein, 9 aa, synthetic construct
GGDGNDDVR

SEQ ID NO: 7164 - protein, 9 aa, synthetic construct
GGAGDDYVS

SEQ ID NO: 7165 - protein, 9 aa, synthetic construct
GGAGRDLLA

SEQ ID NO: 7166 - protein, 9 aa, synthetic construct
GGAGADSII

SEQ ID NO: 7167 - protein, 9 aa, synthetic construct
GGTGRDTII

SEQ ID NO: 7168 - protein, 9 aa, synthetic construct
GGRGDDVLY

SEQ ID NO: 7169 - protein, 9 aa, synthetic construct
GGAGDDYME

SEQ ID NO: 7170 - protein, 9 aa, synthetic construct
GGAGADSLG

SEQ ID NO: 7171 - protein, 9 aa, synthetic construct
GGAGRDELH

SEQ ID NO: 7172 - protein, 9 aa, synthetic construct
GGAGEDLLD

SEQ ID NO: 7173 - protein, 9 aa, synthetic construct
GGLGADSLN

SEQ ID NO: 7174 - protein, 9 aa, synthetic construct
GGAGADRLQ

SEQ ID NO: 7175 - protein, 9 aa, synthetic construct
GGRGNDILE

SEQ ID NO: 7176 - protein, 9 aa, synthetic construct
GGAGEDRLW

SEQ ID NO: 7177 - protein, 9 aa, synthetic construct
GGIGDDRYV

SEQ ID NO: 7178 - protein, 9 aa, synthetic construct
GGAGEDRLN

SEQ ID NO: 7179 - protein, 9 aa, synthetic construct
GGEGHDKLF

SEQ ID NO: 7180 - protein, 9 aa, synthetic construct
GGPGDDRLL

SEQ ID NO: 7181 - protein, 9 aa, synthetic construct
GGAGEDRLF

SEQ ID NO: 7182 - protein, 9 aa, synthetic construct
GGEGCDVLI

SEQ ID NO: 7183 - protein, 9 aa, synthetic construct
GGIGDDRLY

SEQ ID NO: 7184 - protein, 9 aa, synthetic construct
GGAGADRIF

SEQ ID NO: 7185 - protein, 9 aa, synthetic construct
GGPGDDRLY

SEQ ID NO: 7186 - protein, 9 aa, synthetic construct
GGRGNDDLW

SEQ ID NO: 7187 - protein, 9 aa, synthetic construct
GGAGQDVLF

SEQ ID NO: 7188 - protein, 9 aa, synthetic construct
GGGGADIFK

SEQ ID NO: 7189 - protein, 9 aa, synthetic construct
GGRGNDALY

SEQ ID NO: 7190 - protein, 9 aa, synthetic construct
GGDGDDFLR

SEQ ID NO: 7191 - protein, 9 aa, synthetic construct
GGTGQDTIF

SEQ ID NO: 7192 - protein, 9 aa, synthetic construct
GGTGQDTIL

SEQ ID NO: 7193 - protein, 9 aa, synthetic construct
GGAGKDVLI

SEQ ID NO: 7194 - protein, 9 aa, synthetic construct
GGGGVDSIV

SEQ ID NO: 7195 - protein, 9 aa, synthetic construct
GGWGNDLLD

SEQ ID NO: 7196 - protein, 9 aa, synthetic construct
GGPGDDTLR

SEQ ID NO: 7197 - protein, 9 aa, synthetic construct
GGNGHDSLE

SEQ ID NO: 7198 - protein, 9 aa, synthetic construct
GGEGSDTLV

SEQ ID NO: 7199 - protein, 9 aa, synthetic construct
GGLGDDLII

SEQ ID NO: 7200 - protein, 9 aa, synthetic construct
GGLGADDLV

SEQ ID NO: 7201 - protein, 9 aa, synthetic construct
GGDGTDRMQ

SEQ ID NO: 7202 - protein, 9 aa, synthetic construct
GGLGDDVYR

SEQ ID NO: 7203 - protein, 9 aa, synthetic construct
GGEGADQFV

SEQ ID NO: 7204 - protein, 9 aa, synthetic construct
GGHGDDSLI

SEQ ID NO: 7205 - protein, 9 aa, synthetic construct
GGAGDDKLL

SEQ ID NO: 7206 - protein, 9 aa, synthetic construct
GGLGHDMIN

SEQ ID NO: 7207 - protein, 9 aa, synthetic construct
GGGGLDTLN

SEQ ID NO: 7208 - protein, 9 aa, synthetic construct
GGQGGDSIQ

SEQ ID NO: 7209 - protein, 9 aa, synthetic construct
GGEGFDLLD

SEQ ID NO: 7210 - protein, 9 aa, synthetic construct
GGAGSDTIR

SEQ ID NO: 7211 - protein, 9 aa, synthetic construct
GGHGNDLMH

SEQ ID NO: 7212 - protein, 9 aa, synthetic construct
GGAGSDTLG

SEQ ID NO: 7213 - protein, 9 aa, synthetic construct
GGAGSDTMR

SEQ ID NO: 7214 - protein, 9 aa, synthetic construct
GGGGADVLR

SEQ ID NO: 7215 - protein, 9 aa, synthetic construct
GGGGLDTMH

SEQ ID NO: 7216 - protein, 9 aa, synthetic construct
GGQGADAMT

SEQ ID NO: 7217 - protein, 9 aa, synthetic construct
GGNGLDLIF

SEQ ID NO: 7218 - protein, 9 aa, synthetic construct
GGMGNDTLT

SEQ ID NO: 7219 - protein, 9 aa, synthetic construct
GGAGSDTVF

SEQ ID NO: 7220 - protein, 9 aa, synthetic construct
GGQGEDSLF

SEQ ID NO: 7221 - protein, 9 aa, synthetic construct
GGQGADFFV

SEQ ID NO: 7222 - protein, 9 aa, synthetic construct
GGAGDDIMT

SEQ ID NO: 7223 - protein, 9 aa, synthetic construct
GGQGADLLT

SEQ ID NO: 7224 - protein, 9 aa, synthetic construct
GGDGDDVVA

SEQ ID NO: 7225 - protein, 9 aa, synthetic construct
GGQGDDYVN

SEQ ID NO: 7226 - protein, 9 aa, synthetic construct
GGLGDDVYI

SEQ ID NO: 7227 - protein, 9 aa, synthetic construct
GGVGDDYLS

SEQ ID NO: 7228 - protein, 9 aa, synthetic construct
GGVGHDTLY

SEQ ID NO: 7229 - protein, 9 aa, synthetic construct
GGVGDDTLV

SEQ ID NO: 7230 - protein, 9 aa, synthetic construct
GGVGNDVIR

SEQ ID NO: 7231 - protein, 9 aa, synthetic construct
GGAGDDDLD

SEQ ID NO: 7232 - protein, 9 aa, synthetic construct
GGAGSDQFV

SEQ ID NO: 7233 - protein, 9 aa, synthetic construct
GGGGRDSLY

SEQ ID NO: 7234 - protein, 9 aa, synthetic construct
GGGGLDTIR

SEQ ID NO: 7235 - protein, 9 aa, synthetic construct
GGQGNDALY

SEQ ID NO: 7236 - protein, 9 aa, synthetic construct
GGAGSDRID

SEQ ID NO: 7237 - protein, 9 aa, synthetic construct
GGHGNDTLS

SEQ ID NO: 7238 - protein, 9 aa, synthetic construct
GGAGDDLIM

SEQ ID NO: 7239 - protein, 9 aa, synthetic construct
GGPGTDRLY

SEQ ID NO: 7240 - protein, 9 aa, synthetic construct
GGVGDDTLK

SEQ ID NO: 7241 - protein, 9 aa, synthetic construct
GGDGADYIY

SEQ ID NO: 7242 - protein, 9 aa, synthetic construct
GGAGSDSLN

SEQ ID NO: 7243 - protein, 9 aa, synthetic construct
GGAGTDRLT

SEQ ID NO: 7244 - protein, 9 aa, synthetic construct
GGAGSDRMT

SEQ ID NO: 7245 - protein, 9 aa, synthetic construct
GGQGKDSYV

SEQ ID NO: 7246 - protein, 9 aa, synthetic construct
GGGGADVIT

SEQ ID NO: 7247 - protein, 9 aa, synthetic construct
GGVGDDVLF

SEQ ID NO: 7248 - protein, 9 aa, synthetic construct
GGVGNDTIS

SEQ ID NO: 7249 - protein, 9 aa, synthetic construct
GGDGKDALY

SEQ ID NO: 7250 - protein, 9 aa, synthetic construct
GGMGNDVLT

SEQ ID NO: 7251 - protein, 9 aa, synthetic construct
GGAGTDRAI

SEQ ID NO: 7252 - protein, 9 aa, synthetic construct
GGHGNDSLE

SEQ ID NO: 7253 - protein, 9 aa, synthetic construct
GGGGRDLLL

SEQ ID NO: 7254 - protein, 9 aa, synthetic construct
GGEGDDELR

SEQ ID NO: 7255 - protein, 9 aa, synthetic construct
GGVGNDRML

SEQ ID NO: 7256 - protein, 9 aa, synthetic construct
GGDGSDVLD

SEQ ID NO: 7257 - protein, 9 aa, synthetic construct
GGDGTDVLR

SEQ ID NO: 7258 - protein, 9 aa, synthetic construct
GGEGNDTYR

SEQ ID NO: 7259 - protein, 9 aa, synthetic construct
GGQGADRLT

SEQ ID NO: 7260 - protein, 9 aa, synthetic construct
GGAGDDELW

SEQ ID NO: 7261 - protein, 9 aa, synthetic construct
GGQGDDLLI

SEQ ID NO: 7262 - protein, 9 aa, synthetic construct
GGGGNDALF

SEQ ID NO: 7263 - protein, 9 aa, synthetic construct
GGVGNDQLN

SEQ ID NO: 7264 - protein, 9 aa, synthetic construct
GGEGFDSLH

SEQ ID NO: 7265 - protein, 9 aa, synthetic construct
GGEGSDIID

SEQ ID NO: 7266 - protein, 9 aa, synthetic construct
GGQGADTFL

SEQ ID NO: 7267 - protein, 9 aa, synthetic construct
GGAGSDYMR

SEQ ID NO: 7268 - protein, 9 aa, synthetic construct
GGDGDDAID

SEQ ID NO: 7269 - protein, 9 aa, synthetic construct
GGVGNDNID

SEQ ID NO: 7270 - protein, 9 aa, synthetic construct
GGAGDDELK

SEQ ID NO: 7271 - protein, 9 aa, synthetic construct
GGNGNDDLV

SEQ ID NO: 7272 - protein, 9 aa, synthetic construct
GGQGDDIID

SEQ ID NO: 7273 - protein, 9 aa, synthetic construct
GGLGGDTFI

SEQ ID NO: 7274 - protein, 9 aa, synthetic construct
GGQGDDHLY

SEQ ID NO: 7275 - protein, 9 aa, synthetic construct
GGGGNDAIN

SEQ ID NO: 7276 - protein, 9 aa, synthetic construct
GGEGDDFLA

SEQ ID NO: 7277 - protein, 9 aa, synthetic construct
GGEGDDFIN

SEQ ID NO: 7278 - protein, 9 aa, synthetic construct
GGGGDDEIY

SEQ ID NO: 7279 - protein, 9 aa, synthetic construct
GGAGTDELH

SEQ ID NO: 7280 - protein, 9 aa, synthetic construct
GGGGGDTLF

SEQ ID NO: 7281 - protein, 9 aa, synthetic construct
GGGGRDRLI

SEQ ID NO: 7282 - protein, 9 aa, synthetic construct
GGAGDDELL

SEQ ID NO: 7283 - protein, 9 aa, synthetic construct
GGDGKDTLI

SEQ ID NO: 7284 - protein, 9 aa, synthetic construct
GGEGDDELS

SEQ ID NO: 7285 - protein, 9 aa, synthetic construct
GGQGDDTIY

SEQ ID NO: 7286 - protein, 9 aa, synthetic construct
GGQGDDVLR

SEQ ID NO: 7287 - protein, 9 aa, synthetic construct
GGVGIDSVS

SEQ ID NO: 7288 - protein, 9 aa, synthetic construct
GGVGIDTLV

SEQ ID NO: 7289 - protein, 9 aa, synthetic construct
GGDGADYLS

SEQ ID NO: 7290 - protein, 9 aa, synthetic construct
GGGGDDFLN

SEQ ID NO: 7291 - protein, 9 aa, synthetic construct
GGAGTDLLI

SEQ ID NO: 7292 - protein, 9 aa, synthetic construct
GGDGDDALS

SEQ ID NO: 7293 - protein, 9 aa, synthetic construct
GGDGDDALR

SEQ ID NO: 7294 - protein, 9 aa, synthetic construct
GGQGDDTVS

SEQ ID NO: 7295 - protein, 9 aa, synthetic construct
GGMGNDTIT

SEQ ID NO: 7296 - protein, 9 aa, synthetic construct
GGEGDDFLN

SEQ ID NO: 7297 - protein, 9 aa, synthetic construct
GGAGDDHLV

SEQ ID NO: 7298 - protein, 9 aa, synthetic construct
GGDGDDWLI

SEQ ID NO: 7299 - protein, 9 aa, synthetic construct
GGAGDDHLS

SEQ ID NO: 7300 - protein, 9 aa, synthetic construct
GGAGDDELH

SEQ ID NO: 7301 - protein, 9 aa, synthetic construct
GGAGDDHLH

SEQ ID NO: 7302 - protein, 9 aa, synthetic construct
GGQGDDSLL

SEQ ID NO: 7303 - protein, 9 aa, synthetic construct
GGDGTDTIN

SEQ ID NO: 7304 - protein, 9 aa, synthetic construct
GGQGDDSLD

SEQ ID NO: 7305 - protein, 9 aa, synthetic construct
GGDGDDALE

SEQ ID NO: 7306 - protein, 9 aa, synthetic construct
GGDGDDALD

SEQ ID NO: 7307 - protein, 9 aa, synthetic construct
GGMGNDSLY

SEQ ID NO: 7308 - protein, 9 aa, synthetic construct
GGAGDDGLV

SEQ ID NO: 7309 - protein, 9 aa, synthetic construct
GGAGSDVYR

SEQ ID NO: 7310 - protein, 9 aa, synthetic construct
GGMGNDYLN

SEQ ID NO: 7311 - protein, 9 aa, synthetic construct
GGAGDDLVF

SEQ ID NO: 7312 - protein, 9 aa, synthetic construct
GGQGNDILA

SEQ ID NO: 7313 - protein, 9 aa, synthetic construct
GGVGADILD

SEQ ID NO: 7314 - protein, 9 aa, synthetic construct
GGAGSDFAI

SEQ ID NO: 7315 - protein, 9 aa, synthetic construct
GGEGRDVFV

SEQ ID NO: 7316 - protein, 9 aa, synthetic construct
GGAGDDRMD

SEQ ID NO: 7317 - protein, 9 aa, synthetic construct
GGGGRDTLT

SEQ ID NO: 7318 - protein, 9 aa, synthetic construct
GGLGDDNLD

SEQ ID NO: 7319 - protein, 9 aa, synthetic construct
GGNGNDILQ

SEQ ID NO: 7320 - protein, 9 aa, synthetic construct
GGAGDDRIS

SEQ ID NO: 7321 - protein, 9 aa, synthetic construct
GGAGSDFLD

SEQ ID NO: 7322 - protein, 9 aa, synthetic construct
GGDGGDSLY

SEQ ID NO: 7323 - protein, 9 aa, synthetic construct
GGLGDDQLD

SEQ ID NO: 7324 - protein, 9 aa, synthetic construct
GGAGDDRAS

SEQ ID NO: 7325 - protein, 9 aa, synthetic construct
GGLGKDLIY

SEQ ID NO: 7326 - protein, 9 aa, synthetic construct
GGNGNDILT

SEQ ID NO: 7327 - protein, 9 aa, synthetic construct
GGNGNDIFV

SEQ ID NO: 7328 - protein, 9 aa, synthetic construct
GGVGRDTMF

SEQ ID NO: 7329 - protein, 9 aa, synthetic construct
GGAGTDYLY

SEQ ID NO: 7330 - protein, 9 aa, synthetic construct
GGQGQDSLD

SEQ ID NO: 7331 - protein, 9 aa, synthetic construct
GGLGRDKMW

SEQ ID NO: 7332 - protein, 9 aa, synthetic construct
GGLGIDTLT

SEQ ID NO: 7333 - protein, 9 aa, synthetic construct
GGDGDDVFR

SEQ ID NO: 7334 - protein, 9 aa, synthetic construct
GGAGDDQLW

SEQ ID NO: 7335 - protein, 9 aa, synthetic construct
GGEGRDVLT

SEQ ID NO: 7336 - protein, 9 aa, synthetic construct
GGLGDDRLW

SEQ ID NO: 7337 - protein, 9 aa, synthetic construct
GGHGSDTID

SEQ ID NO: 7338 - protein, 9 aa, synthetic construct
GGAGSDEVY

SEQ ID NO: 7339 - protein, 9 aa, synthetic construct
GGTGYDLIR

SEQ ID NO: 7340 - protein, 9 aa, synthetic construct
GGVGDDLYI

SEQ ID NO: 7341 - protein, 9 aa, synthetic construct
GGLGKDTLN

SEQ ID NO: 7342 - protein, 9 aa, synthetic construct
GGDGDDTVT

SEQ ID NO: 7343 - protein, 9 aa, synthetic construct
GGAGDDSIY

SEQ ID NO: 7344 - protein, 9 aa, synthetic construct
GGHGADIMD

SEQ ID NO: 7345 - protein, 9 aa, synthetic construct
GGLGDDLLL

SEQ ID NO: 7346 - protein, 9 aa, synthetic construct
GGPGNDSLL

SEQ ID NO: 7347 - protein, 9 aa, synthetic construct
GGGGADRME

SEQ ID NO: 7348 - protein, 9 aa, synthetic construct
GGLGKDTLS

SEQ ID NO: 7349 - protein, 9 aa, synthetic construct
GGAGDDSIF

SEQ ID NO: 7350 - protein, 9 aa, synthetic construct
GGTGADTMQ

SEQ ID NO: 7351 - protein, 9 aa, synthetic construct
GGLGRDLLT

SEQ ID NO: 7352 - protein, 9 aa, synthetic construct
GGTGVDTMS

SEQ ID NO: 7353 - protein, 9 aa, synthetic construct
GGQGSDTLF

SEQ ID NO: 7354 - protein, 9 aa, synthetic construct
GGAGDDRVD

SEQ ID NO: 7355 - protein, 9 aa, synthetic construct
GGEGSDTLA

SEQ ID NO: 7356 - protein, 9 aa, synthetic construct
GGQGSDTFV

SEQ ID NO: 7357 - protein, 9 aa, synthetic construct
GGLGTDVLD

SEQ ID NO: 7358 - protein, 9 aa, synthetic construct
GGEGSDTIS

SEQ ID NO: 7359 - protein, 9 aa, synthetic construct
GGPGNDTIY

SEQ ID NO: 7360 - protein, 9 aa, synthetic construct
GGGGADSFI

SEQ ID NO: 7361 - protein, 9 aa, synthetic construct
GGAGSDDLQ

SEQ ID NO: 7362 - protein, 9 aa, synthetic construct
GGDGMDFVN

SEQ ID NO: 7363 - protein, 9 aa, synthetic construct
GGLGDDLYY

SEQ ID NO: 7364 - protein, 9 aa, synthetic construct
GGDGDDYLH

SEQ ID NO: 7365 - protein, 9 aa, synthetic construct
GGMGIDTVR

SEQ ID NO: 7366 - protein, 9 aa, synthetic construct
GGAGDDQLL

SEQ ID NO: 7367 - protein, 9 aa, synthetic construct
GGQGNDYID

SEQ ID NO: 7368 - protein, 9 aa, synthetic construct
GGVGADQLF

SEQ ID NO: 7369 - protein, 9 aa, synthetic construct
GGAGDDMLV

SEQ ID NO: 7370 - protein, 9 aa, synthetic construct
GGQGNDSII

SEQ ID NO: 7371 - protein, 9 aa, synthetic construct
GGQGNDSID

SEQ ID NO: 7372 - protein, 9 aa, synthetic construct
GGQGNDRLE

SEQ ID NO: 7373 - protein, 9 aa, synthetic construct
GGVGNDWLS

SEQ ID NO: 7374 - protein, 9 aa, synthetic construct
GGPGSDRFV

SEQ ID NO: 7375 - protein, 9 aa, synthetic construct
GGVGDDELR

SEQ ID NO: 7376 - protein, 9 aa, synthetic construct
GGEGNDTLG

SEQ ID NO: 7377 - protein, 9 aa, synthetic construct
GGGGNDFLA

SEQ ID NO: 7378 - protein, 9 aa, synthetic construct
GGAGTDTFV

SEQ ID NO: 7379 - protein, 9 aa, synthetic construct
GGAGDDMLY

SEQ ID NO: 7380 - protein, 9 aa, synthetic construct
GGAGDDDID

SEQ ID NO: 7381 - protein, 9 aa, synthetic construct
GGVGDDFVA

SEQ ID NO: 7382 - protein, 9 aa, synthetic construct
GGGGNDFLR

SEQ ID NO: 7383 - protein, 9 aa, synthetic construct
GGAGDDMLS

SEQ ID NO: 7384 - protein, 9 aa, synthetic construct
GGQGNDMLS

SEQ ID NO: 7385 - protein, 9 aa, synthetic construct
GGQGNDMLI

SEQ ID NO: 7386 - protein, 9 aa, synthetic construct
GGVGDDILI

SEQ ID NO: 7387 - protein, 9 aa, synthetic construct
GGAGDDMIY

SEQ ID NO: 7388 - protein, 9 aa, synthetic construct
GGQGNDLLV

SEQ ID NO: 7389 - protein, 9 aa, synthetic construct
GGAGTDTAF

SEQ ID NO: 7390 - protein, 9 aa, synthetic construct
GGAGTDTAA

SEQ ID NO: 7391 - protein, 9 aa, synthetic construct
GGVGNDVLD

SEQ ID NO: 7392 - protein, 9 aa, synthetic construct
GGDGDDVLG

SEQ ID NO: 7393 - protein, 9 aa, synthetic construct
GGLGDDTLF

SEQ ID NO: 7394 - protein, 9 aa, synthetic construct
GGGGLDLLL

SEQ ID NO: 7395 - protein, 9 aa, synthetic construct
GGNGKDSFV

SEQ ID NO: 7396 - protein, 9 aa, synthetic construct
GGAGDDNLQ

SEQ ID NO: 7397 - protein, 9 aa, synthetic construct
GGAGDDALV

SEQ ID NO: 7398 - protein, 9 aa, synthetic construct
GGVGRDSLS

SEQ ID NO: 7399 - protein, 9 aa, synthetic construct
GGEGGDRFF

SEQ ID NO: 7400 - protein, 9 aa, synthetic construct
GGVGADRFD

SEQ ID NO: 7401 - protein, 9 aa, synthetic construct
GGVGADRLD

SEQ ID NO: 7402 - protein, 9 aa, synthetic construct
GGAGDDQLE

SEQ ID NO: 7403 - protein, 9 aa, synthetic construct
GGQGNDVLQ

SEQ ID NO: 7404 - protein, 9 aa, synthetic construct
GGAGCDTMI

SEQ ID NO: 7405 - protein, 9 aa, synthetic construct
GGVGADRME

SEQ ID NO: 7406 - protein, 9 aa, synthetic construct
GGGGDDILN

SEQ ID NO: 7407 - protein, 9 aa, synthetic construct
GGDGDDYIH

SEQ ID NO: 7408 - protein, 9 aa, synthetic construct
GGAGDDQIQ

SEQ ID NO: 7409 - protein, 9 aa, synthetic construct
GGDGLDTLI

SEQ ID NO: 7410 - protein, 9 aa, synthetic construct
GGHGSDILN

SEQ ID NO: 7411 - protein, 9 aa, synthetic construct
GGAGDDQIL

SEQ ID NO: 7412 - protein, 9 aa, synthetic construct
GGGGRDILD

SEQ ID NO: 7413 - protein, 9 aa, synthetic construct
GGAGDDQIA

SEQ ID NO: 7414 - protein, 9 aa, synthetic construct
GGGGDDIIT

SEQ ID NO: 7415 - protein, 9 aa, synthetic construct
GGLGDDSIS

SEQ ID NO: 7416 - protein, 9 aa, synthetic construct
GGGGADTLM

SEQ ID NO: 7417 - protein, 9 aa, synthetic construct
GGPGRDTLE

SEQ ID NO: 7418 - protein, 9 aa, synthetic construct
GGVGADVLD

SEQ ID NO: 7419 - protein, 9 aa, synthetic construct
GGQGNDSLT

SEQ ID NO: 7420 - protein, 9 aa, synthetic construct
GGLGDDSLI

SEQ ID NO: 7421 - protein, 9 aa, synthetic construct
GGAGYDTLT

SEQ ID NO: 7422 - protein, 9 aa, synthetic construct
GGDGNDFLF

SEQ ID NO: 7423 - protein, 9 aa, synthetic construct
GGAGQDILT

SEQ ID NO: 7424 - protein, 9 aa, synthetic construct
GGDGNDNID

SEQ ID NO: 7425 - protein, 9 aa, synthetic construct
GGFGADSIL

SEQ ID NO: 7426 - protein, 9 aa, synthetic construct
GGYGNDFLD

SEQ ID NO: 7427 - protein, 9 aa, synthetic construct
GGAGNDRIW

SEQ ID NO: 7428 - protein, 9 aa, synthetic construct
GGYGNDELK

SEQ ID NO: 7429 - protein, 9 aa, synthetic construct
GGIGNDSLI

SEQ ID NO: 7430 - protein, 9 aa, synthetic construct
GGGGNDVMD

SEQ ID NO: 7431 - protein, 9 aa, synthetic construct
GGTGFDQLD

SEQ ID NO: 7432 - protein, 9 aa, synthetic construct
GGYGNDDLK

SEQ ID NO: 7433 - protein, 9 aa, synthetic construct
GGAGGDVLV

SEQ ID NO: 7434 - protein, 9 aa, synthetic construct
GGAGNDRMA

SEQ ID NO: 7435 - protein, 9 aa, synthetic construct
GGTGFDTLN

SEQ ID NO: 7436 - protein, 9 aa, synthetic construct
GGDGADNLS

SEQ ID NO: 7437 - protein, 9 aa, synthetic construct
GGGGSDILN

SEQ ID NO: 7438 - protein, 9 aa, synthetic construct
GGGGSDILS

SEQ ID NO: 7439 - protein, 9 aa, synthetic construct
GGLGNDTIG

SEQ ID NO: 7440 - protein, 9 aa, synthetic construct
GGAGGDTYV

SEQ ID NO: 7441 - protein, 9 aa, synthetic construct
GGDGDDRLH

SEQ ID NO: 7442 - protein, 9 aa, synthetic construct
GGNGSDFLD

SEQ ID NO: 7443 - protein, 9 aa, synthetic construct
GGEGDDYID

SEQ ID NO: 7444 - protein, 9 aa, synthetic construct
GGLGNDTFK

SEQ ID NO: 7445 - protein, 9 aa, synthetic construct
GGIGNDQLN

SEQ ID NO: 7446 - protein, 9 aa, synthetic construct
GGTGGDLLA

SEQ ID NO: 7447 - protein, 9 aa, synthetic construct
GGAGGDTMA

SEQ ID NO: 7448 - protein, 9 aa, synthetic construct
GGAGNDRYV

SEQ ID NO: 7449 - protein, 9 aa, synthetic construct
GGAGNDRIR

SEQ ID NO: 7450 - protein, 9 aa, synthetic construct
GGAGNDRIQ

SEQ ID NO: 7451 - protein, 9 aa, synthetic construct
GGEGRDIFR

SEQ ID NO: 7452 - protein, 9 aa, synthetic construct
GGEGNDKLL

SEQ ID NO: 7453 - protein, 9 aa, synthetic construct
GGYGNDRLL

SEQ ID NO: 7454 - protein, 9 aa, synthetic construct
GGGGSDTLN

SEQ ID NO: 7455 - protein, 9 aa, synthetic construct
GGTGDDYLY

SEQ ID NO: 7456 - protein, 9 aa, synthetic construct
GGIGNDTLA

SEQ ID NO: 7457 - protein, 9 aa, synthetic construct
GGFGADTLL

SEQ ID NO: 7458 - protein, 9 aa, synthetic construct
GGSGDDSLR

SEQ ID NO: 7459 - protein, 9 aa, synthetic construct
GGIGNDTIF

SEQ ID NO: 7460 - protein, 9 aa, synthetic construct
GGSGDDSIL

SEQ ID NO: 7461 - protein, 9 aa, synthetic construct
GGDGNDNIT

SEQ ID NO: 7462 - protein, 9 aa, synthetic construct
GGDGDDIVV

SEQ ID NO: 7463 - protein, 9 aa, synthetic construct
GGYGNDLLY

SEQ ID NO: 7464 - protein, 9 aa, synthetic construct
GGKGNDVIQ

SEQ ID NO: 7465 - protein, 9 aa, synthetic construct
GGFGSDRLN

SEQ ID NO: 7466 - protein, 9 aa, synthetic construct
GGSGDDRLT

SEQ ID NO: 7467 - protein, 9 aa, synthetic construct
GGGGNDVLM

SEQ ID NO: 7468 - protein, 9 aa, synthetic construct
GGGGNDVLQ

SEQ ID NO: 7469 - protein, 9 aa, synthetic construct
GGDGADRID

SEQ ID NO: 7470 - protein, 9 aa, synthetic construct
GGNGRDRAW

SEQ ID NO: 7471 - protein, 9 aa, synthetic construct
GGGGEDILA

SEQ ID NO: 7472 - protein, 9 aa, synthetic construct
GGSGDDRIN

SEQ ID NO: 7473 - protein, 9 aa, synthetic construct
GGSGDDRID

SEQ ID NO: 7474 - protein, 9 aa, synthetic construct
GGSGDDRFS

SEQ ID NO: 7475 - protein, 9 aa, synthetic construct
GGAGNDRII

SEQ ID NO: 7476 - protein, 9 aa, synthetic construct
GGEGADTLK

SEQ ID NO: 7477 - protein, 9 aa, synthetic construct
GGAGGDTLE

SEQ ID NO: 7478 - protein, 9 aa, synthetic construct
GGYGNDSIR

SEQ ID NO: 7479 - protein, 9 aa, synthetic construct
GGMGDDKFI

SEQ ID NO: 7480 - protein, 9 aa, synthetic construct
GGGGDDYLA

SEQ ID NO: 7481 - protein, 9 aa, synthetic construct
GGSGDDDLT

SEQ ID NO: 7482 - protein, 9 aa, synthetic construct
GGSGDDDLD

SEQ ID NO: 7483 - protein, 9 aa, synthetic construct
GGAGADILK

SEQ ID NO: 7484 - protein, 9 aa, synthetic construct
GGEGNDLLA

SEQ ID NO: 7485 - protein, 9 aa, synthetic construct
GGNGSDRLY

SEQ ID NO: 7486 - protein, 9 aa, synthetic construct
GGSGDDALD

SEQ ID NO: 7487 - protein, 9 aa, synthetic construct
GGDGADLIY

SEQ ID NO: 7488 - protein, 9 aa, synthetic construct
GGAGNDSYR

SEQ ID NO: 7489 - protein, 9 aa, synthetic construct
GGDGRDSLY

SEQ ID NO: 7490 - protein, 9 aa, synthetic construct
GGTGHDTLT

SEQ ID NO: 7491 - protein, 9 aa, synthetic construct
GGAGNDTAL

SEQ ID NO: 7492 - protein, 9 aa, synthetic construct
GGDGNDMLR

SEQ ID NO: 7493 - protein, 9 aa, synthetic construct
GGDGRDSVI

SEQ ID NO: 7494 - protein, 9 aa, synthetic construct
GGAGNDTAW

SEQ ID NO: 7495 - protein, 9 aa, synthetic construct
GGIGNDILV

SEQ ID NO: 7496 - protein, 9 aa, synthetic construct
GGDGNDLMY

SEQ ID NO: 7497 - protein, 9 aa, synthetic construct
GGNGSDTII

SEQ ID NO: 7498 - protein, 9 aa, synthetic construct
GGEGADYLD

SEQ ID NO: 7499 - protein, 9 aa, synthetic construct
GGNGSDTYL

SEQ ID NO: 7500 - protein, 9 aa, synthetic construct
GGIGNDIIN

SEQ ID NO: 7501 - protein, 9 aa, synthetic construct
GGTGIDKLS

SEQ ID NO: 7502 - protein, 9 aa, synthetic construct
GGSGADVLD

SEQ ID NO: 7503 - protein, 9 aa, synthetic construct
GGAGGDKLF

SEQ ID NO: 7504 - protein, 9 aa, synthetic construct
GGLGNDSYF

SEQ ID NO: 7505 - protein, 9 aa, synthetic construct
GGSGDDDVN

SEQ ID NO: 7506 - protein, 9 aa, synthetic construct
GGAGNDSML

SEQ ID NO: 7507 - protein, 9 aa, synthetic construct
GGLGSDVLN

SEQ ID NO: 7508 - protein, 9 aa, synthetic construct
GGNGADVLS

SEQ ID NO: 7509 - protein, 9 aa, synthetic construct
GGSGDDILK

SEQ ID NO: 7510 - protein, 9 aa, synthetic construct
GGDGNDMLN

SEQ ID NO: 7511 - protein, 9 aa, synthetic construct
GGSGDDILG

SEQ ID NO: 7512 - protein, 9 aa, synthetic construct
GGSGDDIIG

SEQ ID NO: 7513 - protein, 9 aa, synthetic construct
GGAGNDSFK

SEQ ID NO: 7514 - protein, 9 aa, synthetic construct
GGRGRDFLD

SEQ ID NO: 7515 - protein, 9 aa, synthetic construct
GGLGNDTAV

SEQ ID NO: 7516 - protein, 9 aa, synthetic construct
GGTGGDTLT

SEQ ID NO: 7517 - protein, 9 aa, synthetic construct
GGEGADTLH

SEQ ID NO: 7518 - protein, 9 aa, synthetic construct
GGDGDDRLQ

SEQ ID NO: 7519 - protein, 9 aa, synthetic construct
GGDGADLVY

SEQ ID NO: 7520 - protein, 9 aa, synthetic construct
GGAGNDSIR

SEQ ID NO: 7521 - protein, 9 aa, synthetic construct
GGAGGDSLT

SEQ ID NO: 7522 - protein, 9 aa, synthetic construct
GGDGDDRLR

SEQ ID NO: 7523 - protein, 9 aa, synthetic construct
GGDGNDMLE

SEQ ID NO: 7524 - protein, 9 aa, synthetic construct
GGGGNDWIS

SEQ ID NO: 7525 - protein, 9 aa, synthetic construct
GGIGNDLLV

SEQ ID NO: 7526 - protein, 9 aa, synthetic construct
GGAGGDRMV

SEQ ID NO: 7527 - protein, 9 aa, synthetic construct
GGLGNDSYY

SEQ ID NO: 7528 - protein, 9 aa, synthetic construct
GGSGDDEID

SEQ ID NO: 7529 - protein, 9 aa, synthetic construct
GGAGGDRFI

SEQ ID NO: 7530 - protein, 9 aa, synthetic construct
GGYGHDRMT

SEQ ID NO: 7531 - protein, 9 aa, synthetic construct
GGDGADRLT

SEQ ID NO: 7532 - protein, 9 aa, synthetic construct
GGDGHDILL

SEQ ID NO: 7533 - protein, 9 aa, synthetic construct
GGDGRDTLA

SEQ ID NO: 7534 - protein, 9 aa, synthetic construct
GGDGDDQMF

SEQ ID NO: 7535 - protein, 9 aa, synthetic construct
GGDGNDQLW

SEQ ID NO: 7536 - protein, 9 aa, synthetic construct
GGAGADAMY

SEQ ID NO: 7537 - protein, 9 aa, synthetic construct
GGDGADTLH

SEQ ID NO: 7538 - protein, 9 aa, synthetic construct
GGNGNDTVE

SEQ ID NO: 7539 - protein, 9 aa, synthetic construct
GGNGNDTVI

SEQ ID NO: 7540 - protein, 9 aa, synthetic construct
GGTGDDILL

SEQ ID NO: 7541 - protein, 9 aa, synthetic construct
GGGGNDVFL

SEQ ID NO: 7542 - protein, 9 aa, synthetic construct
GGEGADTMD

SEQ ID NO: 7543 - protein, 9 aa, synthetic construct
GGNGNDTYI

SEQ ID NO: 7544 - protein, 9 aa, synthetic construct
GGSGFDTLI

SEQ ID NO: 7545 - protein, 9 aa, synthetic construct
GGSGFDTLD

SEQ ID NO: 7546 - protein, 9 aa, synthetic construct
GGAGHDRLS

SEQ ID NO: 7547 - protein, 9 aa, synthetic construct
GGNGNDVID

SEQ ID NO: 7548 - protein, 9 aa, synthetic construct
GGAGADDFV

SEQ ID NO: 7549 - protein, 9 aa, synthetic construct
GGAGNDLMR

SEQ ID NO: 7550 - protein, 9 aa, synthetic construct
GGEGQDTLF

SEQ ID NO: 7551 - protein, 9 aa, synthetic construct
GGAGNDLVF

SEQ ID NO: 7552 - protein, 9 aa, synthetic construct
GGTGDDLIF

SEQ ID NO: 7553 - protein, 9 aa, synthetic construct
GGSGFDNIT

SEQ ID NO: 7554 - protein, 9 aa, synthetic construct
GGAGNDLVN

SEQ ID NO: 7555 - protein, 9 aa, synthetic construct
GGAGNDLVS

SEQ ID NO: 7556 - protein, 9 aa, synthetic construct
GGAGHDRIF

SEQ ID NO: 7557 - protein, 9 aa, synthetic construct
GGGGSDLLL

SEQ ID NO: 7558 - protein, 9 aa, synthetic construct
GGSGFDILI

SEQ ID NO: 7559 - protein, 9 aa, synthetic construct
GGKGNDKLV

SEQ ID NO: 7560 - protein, 9 aa, synthetic construct
GGGGSDRLD

SEQ ID NO: 7561 - protein, 9 aa, synthetic construct
GGNGNDTIF

SEQ ID NO: 7562 - protein, 9 aa, synthetic construct
GGNGDDYLS

SEQ ID NO: 7563 - protein, 9 aa, synthetic construct
GGIGSDIFS

SEQ ID NO: 7564 - protein, 9 aa, synthetic construct
GGAGNDIIH

SEQ ID NO: 7565 - protein, 9 aa, synthetic construct
GGTGADVID

SEQ ID NO: 7566 - protein, 9 aa, synthetic construct
GGYGYDRVN

SEQ ID NO: 7567 - protein, 9 aa, synthetic construct
GGAGHDVLH

SEQ ID NO: 7568 - protein, 9 aa, synthetic construct
GGAGHDVLF

SEQ ID NO: 7569 - protein, 9 aa, synthetic construct
GGAGHDVLD

SEQ ID NO: 7570 - protein, 9 aa, synthetic construct
GGTGADWLD

SEQ ID NO: 7571 - protein, 9 aa, synthetic construct
GGGGNDTMY

SEQ ID NO: 7572 - protein, 9 aa, synthetic construct
GGYGWDYLD

SEQ ID NO: 7573 - protein, 9 aa, synthetic construct
GGAGNDIVF

SEQ ID NO: 7574 - protein, 9 aa, synthetic construct
GGAGNDIVN

SEQ ID NO: 7575 - protein, 9 aa, synthetic construct
GGAGNDIVY

SEQ ID NO: 7576 - protein, 9 aa, synthetic construct
GGAGADAFR

SEQ ID NO: 7577 - protein, 9 aa, synthetic construct
GGAGADAFW

SEQ ID NO: 7578 - protein, 9 aa, synthetic construct
GGMGADSLD

SEQ ID NO: 7579 - protein, 9 aa, synthetic construct
GGKGNDHLS

SEQ ID NO: 7580 - protein, 9 aa, synthetic construct
GGSGGDTYV

SEQ ID NO: 7581 - protein, 9 aa, synthetic construct
GGDGDDQLD

SEQ ID NO: 7582 - protein, 9 aa, synthetic construct
GGAGHDTLR

SEQ ID NO: 7583 - protein, 9 aa, synthetic construct
GGLGSDTLK

SEQ ID NO: 7584 - protein, 9 aa, synthetic construct
GGFGDDILN

SEQ ID NO: 7585 - protein, 9 aa, synthetic construct
GGDGDDQLL

SEQ ID NO: 7586 - protein, 9 aa, synthetic construct
GGLGSDILV

SEQ ID NO: 7587 - protein, 9 aa, synthetic construct
GGAGADDIT

SEQ ID NO: 7588 - protein, 9 aa, synthetic construct
GGTGDDYID

SEQ ID NO: 7589 - protein, 9 aa, synthetic construct
GGSGDDTVD

SEQ ID NO: 7590 - protein, 9 aa, synthetic construct
GGTGDDSLA

SEQ ID NO: 7591 - protein, 9 aa, synthetic construct
GGNGNDSLF

SEQ ID NO: 7592 - protein, 9 aa, synthetic construct
GGAGNDQIR

SEQ ID NO: 7593 - protein, 9 aa, synthetic construct
GGTGDDSLI

SEQ ID NO: 7594 - protein, 9 aa, synthetic construct
GGTGDDSMM

SEQ ID NO: 7595 - protein, 9 aa, synthetic construct
GGDGADSLF

SEQ ID NO: 7596 - protein, 9 aa, synthetic construct
GGTGDDTIF

SEQ ID NO: 7597 - protein, 9 aa, synthetic construct
GGIGNDVFV

SEQ ID NO: 7598 - protein, 9 aa, synthetic construct
GGAGNDQLG

SEQ ID NO: 7599 - protein, 9 aa, synthetic construct
GGLGNDVLH

SEQ ID NO: 7600 - protein, 9 aa, synthetic construct
GGTGDDTVK

SEQ ID NO: 7601 - protein, 9 aa, synthetic construct
GGAGNDQMF

SEQ ID NO: 7602 - protein, 9 aa, synthetic construct
GGSGEDYLS

SEQ ID NO: 7603 - protein, 9 aa, synthetic construct
GGTGDDVLQ

SEQ ID NO: 7604 - protein, 9 aa, synthetic construct
GGFGADTVL

SEQ ID NO: 7605 - protein, 9 aa, synthetic construct
GGLGNDVIV

SEQ ID NO: 7606 - protein, 9 aa, synthetic construct
GGLGNDVIN

SEQ ID NO: 7607 - protein, 9 aa, synthetic construct
GGSGDDTIT

SEQ ID NO: 7608 - protein, 9 aa, synthetic construct
GGTGDDVYV

SEQ ID NO: 7609 - protein, 9 aa, synthetic construct
GGSGDDTIA

SEQ ID NO: 7610 - protein, 9 aa, synthetic construct
GGGGSDTLE

SEQ ID NO: 7611 - protein, 9 aa, synthetic construct
GGNGDDAFD

SEQ ID NO: 7612 - protein, 9 aa, synthetic construct
GGTGDDWLS

SEQ ID NO: 7613 - protein, 9 aa, synthetic construct
GGSGDDTAV

SEQ ID NO: 7614 - protein, 9 aa, synthetic construct
GGSGDDVYI

SEQ ID NO: 7615 - protein, 9 aa, synthetic construct
GGSGDDVYL

SEQ ID NO: 7616 - protein, 9 aa, synthetic construct
GGAGADELN

SEQ ID NO: 7617 - protein, 9 aa, synthetic construct
GGTGDDSIE

SEQ ID NO: 7618 - protein, 9 aa, synthetic construct
GGYGSDLLE

SEQ ID NO: 7619 - protein, 9 aa, synthetic construct
GGAGADDLL

SEQ ID NO: 7620 - protein, 9 aa, synthetic construct
GGIGNDYLR

SEQ ID NO: 7621 - protein, 9 aa, synthetic construct
GGNGNDVLK

SEQ ID NO: 7622 - protein, 9 aa, synthetic construct
GGAGHDNIG

SEQ ID NO: 7623 - protein, 9 aa, synthetic construct
GGNGNDVLL

SEQ ID NO: 7624 - protein, 9 aa, synthetic construct
GGIGNDYLE

SEQ ID NO: 7625 - protein, 9 aa, synthetic construct
GGKGNDRLE

SEQ ID NO: 7626 - protein, 9 aa, synthetic construct
GGSGEDKLY

SEQ ID NO: 7627 - protein, 9 aa, synthetic construct
GGAGADELI

SEQ ID NO: 7628 - protein, 9 aa, synthetic construct
GGSGEDILS

SEQ ID NO: 7629 - protein, 9 aa, synthetic construct
GGAGNDNLL

SEQ ID NO: 7630 - protein, 9 aa, synthetic construct
GGAGNDNLR

SEQ ID NO: 7631 - protein, 9 aa, synthetic construct
GGSGEDALF

SEQ ID NO: 7632 - protein, 9 aa, synthetic construct
GGKGNDSLF

SEQ ID NO: 7633 - protein, 9 aa, synthetic construct
GGAGADELL

SEQ ID NO: 7634 - protein, 9 aa, synthetic construct
GGSGDDYLF

SEQ ID NO: 7635 - protein, 9 aa, synthetic construct
GGDGEDTFV

SEQ ID NO: 7636 - protein, 9 aa, synthetic construct
GGLGSDTVT

SEQ ID NO: 7637 - protein, 9 aa, synthetic construct
GGDGDDRAE

SEQ ID NO: 7638 - protein, 9 aa, synthetic construct
GGIGNDVLY

SEQ ID NO: 7639 - protein, 9 aa, synthetic construct
GGNGEDRLN

SEQ ID NO: 7640 - protein, 9 aa, synthetic construct
GGEGDDRLT

SEQ ID NO: 7641 - protein, 9 aa, synthetic construct
GGSGADTVD

SEQ ID NO: 7642 - protein, 9 aa, synthetic construct
GGAGTDFLE

SEQ ID NO: 7643 - protein, 9 aa, synthetic construct
GGDGHDRLF

SEQ ID NO: 7644 - protein, 9 aa, synthetic construct
GGGGSDELR

SEQ ID NO: 7645 - protein, 9 aa, synthetic construct
GGSGADLLF

SEQ ID NO: 7646 - protein, 9 aa, synthetic construct
GGEGVDVLD

SEQ ID NO: 7647 - protein, 9 aa, synthetic construct
GGEGNDYLY

SEQ ID NO: 7648 - protein, 9 aa, synthetic construct
GGAGFDTLY

SEQ ID NO: 7649 - protein, 9 aa, synthetic construct
GGGGHDTLK

SEQ ID NO: 7650 - protein, 9 aa, synthetic construct
GGDGSDIYE

SEQ ID NO: 7651 - protein, 9 aa, synthetic construct
GGFGVDTVI

SEQ ID NO: 7652 - protein, 9 aa, synthetic construct
GGSGADKMF

SEQ ID NO: 7653 - protein, 9 aa, synthetic construct
GGDGADAFR

SEQ ID NO: 7654 - protein, 9 aa, synthetic construct
GGDGSDILN

SEQ ID NO: 7655 - protein, 9 aa, synthetic construct
GGTGMDVMS

SEQ ID NO: 7656 - protein, 9 aa, synthetic construct
GGSGADKFV

SEQ ID NO: 7657 - protein, 9 aa, synthetic construct
GGTGNDKLS

SEQ ID NO: 7658 - protein, 9 aa, synthetic construct
GGAGFDTAD

SEQ ID NO: 7659 - protein, 9 aa, synthetic construct
GGGGNDLLQ

SEQ ID NO: 7660 - protein, 9 aa, synthetic construct
GGTGNDALL

SEQ ID NO: 7661 - protein, 9 aa, synthetic construct
GGDGHDRLD

SEQ ID NO: 7662 - protein, 9 aa, synthetic construct
GGDGRDYLY

SEQ ID NO: 7663 - protein, 9 aa, synthetic construct
GGIGIDTLA

SEQ ID NO: 7664 - protein, 9 aa, synthetic construct
GGDGADVIH

SEQ ID NO: 7665 - protein, 9 aa, synthetic construct
GGRGSDLIN

SEQ ID NO: 7666 - protein, 9 aa, synthetic construct
GGAGGDALD

SEQ ID NO: 7667 - protein, 9 aa, synthetic construct
GGSGADRFD

SEQ ID NO: 7668 - protein, 9 aa, synthetic construct
GGAGNDTYE

SEQ ID NO: 7669 - protein, 9 aa, synthetic construct
GGAGNDTYK

SEQ ID NO: 7670 - protein, 9 aa, synthetic construct
GGAGNDTYM

SEQ ID NO: 7671 - protein, 9 aa, synthetic construct
GGDGNDLIV

SEQ ID NO: 7672 - protein, 9 aa, synthetic construct
GGDGNDLIS

SEQ ID NO: 7673 - protein, 9 aa, synthetic construct
GGKGVDRLI

SEQ ID NO: 7674 - protein, 9 aa, synthetic construct
GGIGDDYLS

SEQ ID NO: 7675 - protein, 9 aa, synthetic construct
GGPGADRME

SEQ ID NO: 7676 - protein, 9 aa, synthetic construct
GGDGDDILC

SEQ ID NO: 7677 - protein, 9 aa, synthetic construct
GGTGNDMLH

SEQ ID NO: 7678 - protein, 9 aa, synthetic construct
GGGGTDTLV

SEQ ID NO: 7679 - protein, 9 aa, synthetic construct
GGDGADFLY

SEQ ID NO: 7680 - protein, 9 aa, synthetic construct
GGSGADLVD

SEQ ID NO: 7681 - protein, 9 aa, synthetic construct
GGLGNDMLD

SEQ ID NO: 7682 - protein, 9 aa, synthetic construct
GGDGNDIIL

SEQ ID NO: 7683 - protein, 9 aa, synthetic construct
GGDGADALF

SEQ ID NO: 7684 - protein, 9 aa, synthetic construct
GGTGNDAVA

SEQ ID NO: 7685 - protein, 9 aa, synthetic construct
GGAGNDYME

SEQ ID NO: 7686 - protein, 9 aa, synthetic construct
GGDGSDILD

SEQ ID NO: 7687 - protein, 9 aa, synthetic construct
GGDGNDIYI

SEQ ID NO: 7688 - protein, 9 aa, synthetic construct
GGYGADYLD

SEQ ID NO: 7689 - protein, 9 aa, synthetic construct
GGEGNDQLH

SEQ ID NO: 7690 - protein, 9 aa, synthetic construct
GGTGNDELD

SEQ ID NO: 7691 - protein, 9 aa, synthetic construct
GGTGNDELY

SEQ ID NO: 7692 - protein, 9 aa, synthetic construct
GGLGRDYLT

SEQ ID NO: 7693 - protein, 9 aa, synthetic construct
GGGGDDVIN

SEQ ID NO: 7694 - protein, 9 aa, synthetic construct
GGAGFDRID

SEQ ID NO: 7695 - protein, 9 aa, synthetic construct
GGYGADTVL

SEQ ID NO: 7696 - protein, 9 aa, synthetic construct
GGSGADDLY

SEQ ID NO: 7697 - protein, 9 aa, synthetic construct
GGTGNDFLG

SEQ ID NO: 7698 - protein, 9 aa, synthetic construct
GGGGDDVIL

SEQ ID NO: 7699 - protein, 9 aa, synthetic construct
GGDGDDIIA

SEQ ID NO: 7700 - protein, 9 aa, synthetic construct
GGDGNDKLF

SEQ ID NO: 7701 - protein, 9 aa, synthetic construct
GGSGADALF

SEQ ID NO: 7702 - protein, 9 aa, synthetic construct
GGDGADDLI

SEQ ID NO: 7703 - protein, 9 aa, synthetic construct
GGAGNDWLF

SEQ ID NO: 7704 - protein, 9 aa, synthetic construct
GGTGIDTLT

SEQ ID NO: 7705 - protein, 9 aa, synthetic construct
GGAGNDVVT

SEQ ID NO: 7706 - protein, 9 aa, synthetic construct
GGDGADALY

SEQ ID NO: 7707 - protein, 9 aa, synthetic construct
GGLGYDSLT

SEQ ID NO: 7708 - protein, 9 aa, synthetic construct
GGLGNDQLR

SEQ ID NO: 7709 - protein, 9 aa, synthetic construct
GGTGNDIYF

SEQ ID NO: 7710 - protein, 9 aa, synthetic construct
GGSGADIIT

SEQ ID NO: 7711 - protein, 9 aa, synthetic construct
GGDGADELI

SEQ ID NO: 7712 - protein, 9 aa, synthetic construct
GGAGNDYLK

SEQ ID NO: 7713 - protein, 9 aa, synthetic construct
GGYGDDHLD

SEQ ID NO: 7714 - protein, 9 aa, synthetic construct
GGNGGDILF

SEQ ID NO: 7715 - protein, 9 aa, synthetic construct
GGTGNDILE

SEQ ID NO: 7716 - protein, 9 aa, synthetic construct
GGDGADALV

SEQ ID NO: 7717 - protein, 9 aa, synthetic construct
GGDGADALH

SEQ ID NO: 7718 - protein, 9 aa, synthetic construct
GGSGADHLI

SEQ ID NO: 7719 - protein, 9 aa, synthetic construct
GGAGNDYIS

SEQ ID NO: 7720 - protein, 9 aa, synthetic construct
GGAGNDVVD

SEQ ID NO: 7721 - protein, 9 aa, synthetic construct
GGGGDDVIS

SEQ ID NO: 7722 - protein, 9 aa, synthetic construct
GGPGADLLS

SEQ ID NO: 7723 - protein, 9 aa, synthetic construct
GGTGNDIIT

SEQ ID NO: 7724 - protein, 9 aa, synthetic construct
GGPGADSFI

SEQ ID NO: 7725 - protein, 9 aa, synthetic construct
GGSGADAFV

SEQ ID NO: 7726 - protein, 9 aa, synthetic construct
GGGGNDYLE

SEQ ID NO: 7727 - protein, 9 aa, synthetic construct
GGSGADSLK

SEQ ID NO: 7728 - protein, 9 aa, synthetic construct
GGAGGDDID

SEQ ID NO: 7729 - protein, 9 aa, synthetic construct
GGSGADSLE

SEQ ID NO: 7730 - protein, 9 aa, synthetic construct
GGAGADMMI

SEQ ID NO: 7731 - protein, 9 aa, synthetic construct
GGAGNDTVR

SEQ ID NO: 7732 - protein, 9 aa, synthetic construct
GGKGVDTLT

SEQ ID NO: 7733 - protein, 9 aa, synthetic construct
GGGGVDDID

SEQ ID NO: 7734 - protein, 9 aa, synthetic construct
GGDGDDRVS

SEQ ID NO: 7735 - protein, 9 aa, synthetic construct
GGTGNDQLR

SEQ ID NO: 7736 - protein, 9 aa, synthetic construct
GGIGNDALF

SEQ ID NO: 7737 - protein, 9 aa, synthetic construct
GGNGGDTLE

SEQ ID NO: 7738 - protein, 9 aa, synthetic construct
GGEGNDLVY

SEQ ID NO: 7739 - protein, 9 aa, synthetic construct
GGAGADKLH

SEQ ID NO: 7740 - protein, 9 aa, synthetic construct
GGRGRDLIS

SEQ ID NO: 7741 - protein, 9 aa, synthetic construct
GGTGKDTFR

SEQ ID NO: 7742 - protein, 9 aa, synthetic construct
GGAGGDIFL

SEQ ID NO: 7743 - protein, 9 aa, synthetic construct
GGRGRDQLW

SEQ ID NO: 7744 - protein, 9 aa, synthetic construct
GGPGADVLD

SEQ ID NO: 7745 - protein, 9 aa, synthetic construct
GGIGDDVLF

SEQ ID NO: 7746 - protein, 9 aa, synthetic construct
GGSGADTFY

SEQ ID NO: 7747 - protein, 9 aa, synthetic construct
GGNGADTIY

SEQ ID NO: 7748 - protein, 9 aa, synthetic construct
GGNGNDRLH

SEQ ID NO: 7749 - protein, 9 aa, synthetic construct
GGDGNDHLT

SEQ ID NO: 7750 - protein, 9 aa, synthetic construct
GGEGYDFIA

SEQ ID NO: 7751 - protein, 9 aa, synthetic construct
GGYGDDVIH

SEQ ID NO: 7752 - protein, 9 aa, synthetic construct
GGDGADILK

SEQ ID NO: 7753 - protein, 9 aa, synthetic construct
GGNGADTLV

SEQ ID NO: 7754 - protein, 9 aa, synthetic construct
GGEGDDTVN

SEQ ID NO: 7755 - protein, 9 aa, synthetic construct
GGPGADSLL

SEQ ID NO: 7756 - protein, 9 aa, synthetic construct
GGDGADILG

SEQ ID NO: 7757 - protein, 9 aa, synthetic construct
GGGGNDLIN

SEQ ID NO: 7758 - protein, 9 aa, synthetic construct
GGAGADNMQ

SEQ ID NO: 7759 - protein, 9 aa, synthetic construct
GGKGYDILI

SEQ ID NO: 7760 - protein, 9 aa, synthetic construct
GGDGDDHLF

SEQ ID NO: 7761 - protein, 9 aa, synthetic construct
GGGGADALF

SEQ ID NO: 7762 - protein, 9 aa, synthetic construct
GGSGADRIE

SEQ ID NO: 7763 - protein, 9 aa, synthetic construct
GGPGADTLE

SEQ ID NO: 7764 - protein, 9 aa, synthetic construct
GGIGKDWLE

SEQ ID NO: 7765 - protein, 9 aa, synthetic construct
GGSGADSLN

SEQ ID NO: 7766 - protein, 9 aa, synthetic construct
GGAGGDFLY

SEQ ID NO: 7767 - protein, 9 aa, synthetic construct
GGSGADSLY

SEQ ID NO: 7768 - protein, 9 aa, synthetic construct
GGDGSDLIY

SEQ ID NO: 7769 - protein, 9 aa, synthetic construct
GGAGGDIFA

SEQ ID NO: 7770 - protein, 9 aa, synthetic construct
GGDGDDSVF

SEQ ID NO: 7771 - protein, 9 aa, synthetic construct
GGTGKDVFI

SEQ ID NO: 7772 - protein, 9 aa, synthetic construct
GGAGKDVLN

SEQ ID NO: 7773 - protein, 9 aa, synthetic construct
GGLGNDNLA

SEQ ID NO: 7774 - protein, 9 aa, synthetic construct
GGDGNDVII

SEQ ID NO: 7775 - protein, 9 aa, synthetic construct
GGDGADALL

SEQ ID NO: 7776 - protein, 9 aa, synthetic construct
GGLGNDIIN

SEQ ID NO: 7777 - protein, 9 aa, synthetic construct
GGAGTDRLL

SEQ ID NO: 7778 - protein, 9 aa, synthetic construct
GGKGDDTLV

SEQ ID NO: 7779 - protein, 9 aa, synthetic construct
GGAGTDRLS

SEQ ID NO: 7780 - protein, 9 aa, synthetic construct
GGPGDDLLF

SEQ ID NO: 7781 - protein, 9 aa, synthetic construct
GGNGNDQLW

SEQ ID NO: 7782 - protein, 9 aa, synthetic construct
GGNGNDYLR

SEQ ID NO: 7783 - protein, 9 aa, synthetic construct
GGLGNDLIY

SEQ ID NO: 7784 - protein, 9 aa, synthetic construct
GGNGYDYLN

SEQ ID NO: 7785 - protein, 9 aa, synthetic construct
GGLGHDTME

SEQ ID NO: 7786 - protein, 9 aa, synthetic construct
GGSGRDEVY

SEQ ID NO: 7787 - protein, 9 aa, synthetic construct
GGPGSDWLE

SEQ ID NO: 7788 - protein, 9 aa, synthetic construct
GGSGNDTIR

SEQ ID NO: 7789 - protein, 9 aa, synthetic construct
GGGGDDVFV

SEQ ID NO: 7790 - protein, 9 aa, synthetic construct
GGKGDDLLT

SEQ ID NO: 7791 - protein, 9 aa, synthetic construct
GGLGHDTMD

SEQ ID NO: 7792 - protein, 9 aa, synthetic construct
GGDGADSVD

SEQ ID NO: 7793 - protein, 9 aa, synthetic construct
GGPGDDRLW

SEQ ID NO: 7794 - protein, 9 aa, synthetic construct
GGNGNDSVL

SEQ ID NO: 7795 - protein, 9 aa, synthetic construct
GGAGTDSIL

SEQ ID NO: 7796 - protein, 9 aa, synthetic construct
GGLGNDLIL

SEQ ID NO: 7797 - protein, 9 aa, synthetic construct
GGFGNDFIL

SEQ ID NO: 7798 - protein, 9 aa, synthetic construct
GGGGIDTAV

SEQ ID NO: 7799 - protein, 9 aa, synthetic construct
GGQGADVFV

SEQ ID NO: 7800 - protein, 9 aa, synthetic construct
GGDGDDLLG

SEQ ID NO: 7801 - protein, 9 aa, synthetic construct
GGDGGDVLR

SEQ ID NO: 7802 - protein, 9 aa, synthetic construct
GGAGTDSAS

SEQ ID NO: 7803 - protein, 9 aa, synthetic construct
GGAGTDRAV

SEQ ID NO: 7804 - protein, 9 aa, synthetic construct
GGNGNDYLV

SEQ ID NO: 7805 - protein, 9 aa, synthetic construct
GGLGNDLLF

SEQ ID NO: 7806 - protein, 9 aa, synthetic construct
GGDGNDVFY

SEQ ID NO: 7807 - protein, 9 aa, synthetic construct
GGGGDDTIN

SEQ ID NO: 7808 - protein, 9 aa, synthetic construct
GGAGTDILT

SEQ ID NO: 7809 - protein, 9 aa, synthetic construct
GGPGDDNLR

SEQ ID NO: 7810 - protein, 9 aa, synthetic construct
GGAGTDRAS

SEQ ID NO: 7811 - protein, 9 aa, synthetic construct
GGPGDDLLS

SEQ ID NO: 7812 - protein, 9 aa, synthetic construct
GGNGNDVIA

SEQ ID NO: 7813 - protein, 9 aa, synthetic construct
GGNGNDNLS

SEQ ID NO: 7814 - protein, 9 aa, synthetic construct
GGAGTDNLN

SEQ ID NO: 7815 - protein, 9 aa, synthetic construct
GGEGDDFLY

SEQ ID NO: 7816 - protein, 9 aa, synthetic construct
GGEGFDRAL

SEQ ID NO: 7817 - protein, 9 aa, synthetic construct
GGQGADRLF

SEQ ID NO: 7818 - protein, 9 aa, synthetic construct
GGAGLDLLL

SEQ ID NO: 7819 - protein, 9 aa, synthetic construct
GGDGADSIY

SEQ ID NO: 7820 - protein, 9 aa, synthetic construct
GGEGEDHFV

SEQ ID NO: 7821 - protein, 9 aa, synthetic construct
GGEGDDFLR

SEQ ID NO: 7822 - protein, 9 aa, synthetic construct
GGLGNDKLK

SEQ ID NO: 7823 - protein, 9 aa, synthetic construct
GGNGNDTIE

SEQ ID NO: 7824 - protein, 9 aa, synthetic construct
GGLGGDVLR

SEQ ID NO: 7825 - protein, 9 aa, synthetic construct
GGQGADNFV

SEQ ID NO: 7826 - protein, 9 aa, synthetic construct
GGPGDDLLL

SEQ ID NO: 7827 - protein, 9 aa, synthetic construct
GGKGDDKLI

SEQ ID NO: 7828 - protein, 9 aa, synthetic construct
GGQGADRLA

SEQ ID NO: 7829 - protein, 9 aa, synthetic construct
GGNGNDNLI

SEQ ID NO: 7830 - protein, 9 aa, synthetic construct
GGPGADTFV

SEQ ID NO: 7831 - protein, 9 aa, synthetic construct
GGLGQDTLV

SEQ ID NO: 7832 - protein, 9 aa, synthetic construct
GGQGADQLW

SEQ ID NO: 7833 - protein, 9 aa, synthetic construct
GGKGDDTLH

SEQ ID NO: 7834 - protein, 9 aa, synthetic construct
GGPGDDLLY

SEQ ID NO: 7835 - protein, 9 aa, synthetic construct
GGAGLDRLW

SEQ ID NO: 7836 - protein, 9 aa, synthetic construct
GGLGHDNIG

SEQ ID NO: 7837 - protein, 9 aa, synthetic construct
GGNGNDFLA

SEQ ID NO: 7838 - protein, 9 aa, synthetic construct
GGLGGDLLD

SEQ ID NO: 7839 - protein, 9 aa, synthetic construct
GGGGEDRLD

SEQ ID NO: 7840 - protein, 9 aa, synthetic construct
GGSGNDTMF

SEQ ID NO: 7841 - protein, 9 aa, synthetic construct
GGLGGDTLV

SEQ ID NO: 7842 - protein, 9 aa, synthetic construct
GGSGRDLLV

SEQ ID NO: 7843 - protein, 9 aa, synthetic construct
GGDGHDHLY

SEQ ID NO: 7844 - protein, 9 aa, synthetic construct
GGDGADTFL

SEQ ID NO: 7845 - protein, 9 aa, synthetic construct
GGNGNDWIE

SEQ ID NO: 7846 - protein, 9 aa, synthetic construct
GGPGYDTID

SEQ ID NO: 7847 - protein, 9 aa, synthetic construct
GGLGHDLLY

SEQ ID NO: 7848 - protein, 9 aa, synthetic construct
GGDGADTIE

SEQ ID NO: 7849 - protein, 9 aa, synthetic construct
GGQGADRLL

SEQ ID NO: 7850 - protein, 9 aa, synthetic construct
GGLGNDYLI

SEQ ID NO: 7851 - protein, 9 aa, synthetic construct
GGSGRDLLN

SEQ ID NO: 7852 - protein, 9 aa, synthetic construct
GGNGNDEIH

SEQ ID NO: 7853 - protein, 9 aa, synthetic construct
GGPGADVLR

SEQ ID NO: 7854 - protein, 9 aa, synthetic construct
GGGGIDTVS

SEQ ID NO: 7855 - protein, 9 aa, synthetic construct
GGQGADALV

SEQ ID NO: 7856 - protein, 9 aa, synthetic construct
GGNGDDSLE

SEQ ID NO: 7857 - protein, 9 aa, synthetic construct
GGDGADTLM

SEQ ID NO: 7858 - protein, 9 aa, synthetic construct
GGDGNDVIG

SEQ ID NO: 7859 - protein, 9 aa, synthetic construct
GGAGKDVLR

SEQ ID NO: 7860 - protein, 9 aa, synthetic construct
GGDGHDLLE

SEQ ID NO: 7861 - protein, 9 aa, synthetic construct
GGFGNDDLS

SEQ ID NO: 7862 - protein, 9 aa, synthetic construct
GGEGLDVFV

SEQ ID NO: 7863 - protein, 9 aa, synthetic construct
GGDGDDLLK

SEQ ID NO: 7864 - protein, 9 aa, synthetic construct
GGNGSDIYH

SEQ ID NO: 7865 - protein, 9 aa, synthetic construct
GGPGNDRMI

SEQ ID NO: 7866 - protein, 9 aa, synthetic construct
GGPGNDRLW

SEQ ID NO: 7867 - protein, 9 aa, synthetic construct
GGLGNDDLT

SEQ ID NO: 7868 - protein, 9 aa, synthetic construct
GGNGSDIYY

SEQ ID NO: 7869 - protein, 9 aa, synthetic construct
GGSGNDWLS

SEQ ID NO: 7870 - protein, 9 aa, synthetic construct
GGLGNDRLA

SEQ ID NO: 7871 - protein, 9 aa, synthetic construct
GGFGNDIYI

SEQ ID NO: 7872 - protein, 9 aa, synthetic construct
GGDGADTYV

SEQ ID NO: 7873 - protein, 9 aa, synthetic construct
GGAGVDTMV

SEQ ID NO: 7874 - protein, 9 aa, synthetic construct
GGPGNDRIY

SEQ ID NO: 7875 - protein, 9 aa, synthetic construct
GGLGKDVLI

SEQ ID NO: 7876 - protein, 9 aa, synthetic construct
GGEGDDKLF

SEQ ID NO: 7877 - protein, 9 aa, synthetic construct
GGAGVDTMS

SEQ ID NO: 7878 - protein, 9 aa, synthetic construct
GGPGNDLLI

SEQ ID NO: 7879 - protein, 9 aa, synthetic construct
GGAGVDTVQ

SEQ ID NO: 7880 - protein, 9 aa, synthetic construct
GGPGGDILD

SEQ ID NO: 7881 - protein, 9 aa, synthetic construct
GGNGSDILD

SEQ ID NO: 7882 - protein, 9 aa, synthetic construct
GGLGNDTFQ

SEQ ID NO: 7883 - protein, 9 aa, synthetic construct
GGKGDDRLS

SEQ ID NO: 7884 - protein, 9 aa, synthetic construct
GGDGADFLN

SEQ ID NO: 7885 - protein, 9 aa, synthetic construct
GGPGNDTLH

SEQ ID NO: 7886 - protein, 9 aa, synthetic construct
GGLGNDRIE

SEQ ID NO: 7887 - protein, 9 aa, synthetic construct
GGLGNDTFR

SEQ ID NO: 7888 - protein, 9 aa, synthetic construct
GGPGNDTLF

SEQ ID NO: 7889 - protein, 9 aa, synthetic construct
GGLGNDELH

SEQ ID NO: 7890 - protein, 9 aa, synthetic construct
GGPGNDSLF

SEQ ID NO: 7891 - protein, 9 aa, synthetic construct
GGAGVDILV

SEQ ID NO: 7892 - protein, 9 aa, synthetic construct
GGGGDDYLW

SEQ ID NO: 7893 - protein, 9 aa, synthetic construct
GGNGSDIID

SEQ ID NO: 7894 - protein, 9 aa, synthetic construct
GGLGNDELF

SEQ ID NO: 7895 - protein, 9 aa, synthetic construct
GGNGNDLLH

SEQ ID NO: 7896 - protein, 9 aa, synthetic construct
GGAGVDTYY

SEQ ID NO: 7897 - protein, 9 aa, synthetic construct
GGPGGDTAL

SEQ ID NO: 7898 - protein, 9 aa, synthetic construct
GGSGNDWLF

SEQ ID NO: 7899 - protein, 9 aa, synthetic construct
GGPGNDTLQ

SEQ ID NO: 7900 - protein, 9 aa, synthetic construct
GGDGADLVR

SEQ ID NO: 7901 - protein, 9 aa, synthetic construct
GGAGVDTIA

SEQ ID NO: 7902 - protein, 9 aa, synthetic construct
GGGGDDYIE

SEQ ID NO: 7903 - protein, 9 aa, synthetic construct
GGAGVDRLV

SEQ ID NO: 7904 - protein, 9 aa, synthetic construct
GGAGVDRME

SEQ ID NO: 7905 - protein, 9 aa, synthetic construct
GGAGVDRMV

SEQ ID NO: 7906 - protein, 9 aa, synthetic construct
GGAGVDTFK

SEQ ID NO: 7907 - protein, 9 aa, synthetic construct
GGNGTDLAN

SEQ ID NO: 7908 - protein, 9 aa, synthetic construct
GGEGDDYLA

SEQ ID NO: 7909 - protein, 9 aa, synthetic construct
GGLGNDSIV

SEQ ID NO: 7910 - protein, 9 aa, synthetic construct
GGLGNDSIN

SEQ ID NO: 7911 - protein, 9 aa, synthetic construct
GGNGNDRLQ

SEQ ID NO: 7912 - protein, 9 aa, synthetic construct
GGGGKDSLD

SEQ ID NO: 7913 - protein, 9 aa, synthetic construct
GGSGNDVVI

SEQ ID NO: 7914 - protein, 9 aa, synthetic construct
GGAGVDSLS

SEQ ID NO: 7915 - protein, 9 aa, synthetic construct
GGPGIDTLI

SEQ ID NO: 7916 - protein, 9 aa, synthetic construct
GGNGSDTLT

SEQ ID NO: 7917 - protein, 9 aa, synthetic construct
GGSGQDTLY

SEQ ID NO: 7918 - protein, 9 aa, synthetic construct
GGAGVDRLF

SEQ ID NO: 7919 - protein, 9 aa, synthetic construct
GGAGVDTIR

SEQ ID NO: 7920 - protein, 9 aa, synthetic construct
GGDGHDVLD

SEQ ID NO: 7921 - protein, 9 aa, synthetic construct
GGNGNDLIV

SEQ ID NO: 7922 - protein, 9 aa, synthetic construct
GGAGVDTLY

SEQ ID NO: 7923 - protein, 9 aa, synthetic construct
GGAGLDTAS

SEQ ID NO: 7924 - protein, 9 aa, synthetic construct
GGPGNDILR

SEQ ID NO: 7925 - protein, 9 aa, synthetic construct
GGAGVDTLF

SEQ ID NO: 7926 - protein, 9 aa, synthetic construct
GGNGSDRLF

SEQ ID NO: 7927 - protein, 9 aa, synthetic construct
GGPGLDTLH

SEQ ID NO: 7928 - protein, 9 aa, synthetic construct
GGDGHDVVF

SEQ ID NO: 7929 - protein, 9 aa, synthetic construct
GGPGNDALD

SEQ ID NO: 7930 - protein, 9 aa, synthetic construct
GGSGQDTVS

SEQ ID NO: 7931 - protein, 9 aa, synthetic construct
GGNGTDSAS

SEQ ID NO: 7932 - protein, 9 aa, synthetic construct
GGDGADIIY

SEQ ID NO: 7933 - protein, 9 aa, synthetic construct
GGDGADLIV

SEQ ID NO: 7934 - protein, 9 aa, synthetic construct
GGLGNDTIR

SEQ ID NO: 7935 - protein, 9 aa, synthetic construct
GGPGNDTLV

SEQ ID NO: 7936 - protein, 9 aa, synthetic construct
GGGGDDIFA

SEQ ID NO: 7937 - protein, 9 aa, synthetic construct
GGGGDDILE

SEQ ID NO: 7938 - protein, 9 aa, synthetic construct
GGDGHDQLF

SEQ ID NO: 7939 - protein, 9 aa, synthetic construct
GGDGIDTLV

SEQ ID NO: 7940 - protein, 9 aa, synthetic construct
GGDGIDTLI

SEQ ID NO: 7941 - protein, 9 aa, synthetic construct
GGNGDDSLV

SEQ ID NO: 7942 - protein, 9 aa, synthetic construct
GGDGIDTLF

SEQ ID NO: 7943 - protein, 9 aa, synthetic construct
GGDGADRLR

SEQ ID NO: 7944 - protein, 9 aa, synthetic construct
GGLGNDTVS

SEQ ID NO: 7945 - protein, 9 aa, synthetic construct
GGPGRDTFV

SEQ ID NO: 7946 - protein, 9 aa, synthetic construct
GGDGADWVR

SEQ ID NO: 7947 - protein, 9 aa, synthetic construct
GGGGEDTID

SEQ ID NO: 7948 - protein, 9 aa, synthetic construct
GGDGHDTLK

SEQ ID NO: 7949 - protein, 9 aa, synthetic construct
GGNGRDMLS

SEQ ID NO: 7950 - protein, 9 aa, synthetic construct
GGGGDDRLN

SEQ ID NO: 7951 - protein, 9 aa, synthetic construct
GGPGDDVLL

SEQ ID NO: 7952 - protein, 9 aa, synthetic construct
GGNGDDTID

SEQ ID NO: 7953 - protein, 9 aa, synthetic construct
GGPGSDIFV

SEQ ID NO: 7954 - protein, 9 aa, synthetic construct
GGLGNDVFR

SEQ ID NO: 7955 - protein, 9 aa, synthetic construct
GGPGSDILD

SEQ ID NO: 7956 - protein, 9 aa, synthetic construct
GGAGTDTAT

SEQ ID NO: 7957 - protein, 9 aa, synthetic construct
GGDGADSIV

SEQ ID NO: 7958 - protein, 9 aa, synthetic construct
GGNGNDMLD

SEQ ID NO: 7959 - protein, 9 aa, synthetic construct
GGSGNDTVV

SEQ ID NO: 7960 - protein, 9 aa, synthetic construct
GGPGDDSLD

SEQ ID NO: 7961 - protein, 9 aa, synthetic construct
GGLGHDYLD

SEQ ID NO: 7962 - protein, 9 aa, synthetic construct
GGPGDDSLT

SEQ ID NO: 7963 - protein, 9 aa, synthetic construct
GGDGHDTID

SEQ ID NO: 7964 - protein, 9 aa, synthetic construct
GGAGTDTLK

SEQ ID NO: 7965 - protein, 9 aa, synthetic construct
GGGGDDVIF

SEQ ID NO: 7966 - protein, 9 aa, synthetic construct
GGDGADSIE

SEQ ID NO: 7967 - protein, 9 aa, synthetic construct
GGDGNDVVA

SEQ ID NO: 7968 - protein, 9 aa, synthetic construct
GGPGDDTLT

SEQ ID NO: 7969 - protein, 9 aa, synthetic construct
GGNGQDVLN

SEQ ID NO: 7970 - protein, 9 aa, synthetic construct
GGAGLDTLS

SEQ ID NO: 7971 - protein, 9 aa, synthetic construct
GGPGRDLLE

SEQ ID NO: 7972 - protein, 9 aa, synthetic construct
GGGGDDILF

SEQ ID NO: 7973 - protein, 9 aa, synthetic construct
GGPGNDTLY

SEQ ID NO: 7974 - protein, 9 aa, synthetic construct
GGGGDDVIT

SEQ ID NO: 7975 - protein, 9 aa, synthetic construct
GGDGIDTAI

SEQ ID NO: 7976 - protein, 9 aa, synthetic construct
GGNGNDIIS

SEQ ID NO: 7977 - protein, 9 aa, synthetic construct
GGNGNDIIY

SEQ ID NO: 7978 - protein, 9 aa, synthetic construct
GGGGDDLIA

SEQ ID NO: 7979 - protein, 9 aa, synthetic construct
GGGGDDRIE

SEQ ID NO: 7980 - protein, 9 aa, synthetic construct
GGDGADELY

SEQ ID NO: 7981 - protein, 9 aa, synthetic construct
GGPGNDVLY

SEQ ID NO: 7982 - protein, 9 aa, synthetic construct
GGGGKDVLR

SEQ ID NO: 7983 - protein, 9 aa, synthetic construct
GGNGRDVLS

SEQ ID NO: 7984 - protein, 9 aa, synthetic construct
GGLGNDFIM

SEQ ID NO: 7985 - protein, 9 aa, synthetic construct
GGDGADQID

SEQ ID NO: 7986 - protein, 9 aa, synthetic construct
GGGGDDVLE

SEQ ID NO: 7987 - protein, 9 aa, synthetic construct
GGGGDDVLN

SEQ ID NO: 7988 - protein, 9 aa, synthetic construct
GGLGKDSLY

SEQ ID NO: 7989 - protein, 9 aa, synthetic construct
GGGGDDLIS

SEQ ID NO: 7990 - protein, 9 aa, synthetic construct
GGLGNDTLW

SEQ ID NO: 7991 - protein, 9 aa, synthetic construct
GGNGWDTLR

SEQ ID NO: 7992 - protein, 9 aa, synthetic construct
GGLGIDTMI

SEQ ID NO: 7993 - protein, 9 aa, synthetic construct
GGDGADRFI

SEQ ID NO: 7994 - protein, 9 aa, synthetic construct
GGFGNDILN

SEQ ID NO: 7995 - protein, 9 aa, synthetic construct
GGDGHDTLN

SEQ ID NO: 7996 - protein, 9 aa, synthetic construct
GGLGIDTLL

SEQ ID NO: 7997 - protein, 9 aa, synthetic construct
GGNGDDSLY

SEQ ID NO: 7998 - protein, 9 aa, synthetic construct
GGLGNDTVQ

SEQ ID NO: 7999 - protein, 9 aa, synthetic construct
GGNGRDRLI

SEQ ID NO: 8000 - protein, 9 aa, synthetic construct
GGSGQDSLS

SEQ ID NO: 8001 - protein, 9 aa, synthetic construct
GGNGRDTID

SEQ ID NO: 8002 - protein, 9 aa, synthetic construct
GGLGNDTMS

SEQ ID NO: 8003 - protein, 9 aa, synthetic construct
GGLGNDTMN

SEQ ID NO: 8004 - protein, 9 aa, synthetic construct
GGLGNDFLY

SEQ ID NO: 8005 - protein, 9 aa, synthetic construct
GGLGNDTML

SEQ ID NO: 8006 - protein, 9 aa, synthetic construct
GGDGADVLT

SEQ ID NO: 8007 - protein, 9 aa, synthetic construct
GGLGNDTMI

SEQ ID NO: 8008 - protein, 9 aa, synthetic construct
GGGGEDTLT

SEQ ID NO: 8009 - protein, 9 aa, synthetic construct
GGAGNDIFT

SEQ ID NO: 8010 - protein, 9 aa, synthetic construct
GGGGDDDLS

SEQ ID NO: 8011 - protein, 9 aa, synthetic construct
GGSGADAMH

SEQ ID NO: 8012 - protein, 9 aa, synthetic construct
GGAGNDVMA

SEQ ID NO: 8013 - protein, 9 aa, synthetic construct
GGAGNDVME

SEQ ID NO: 8014 - protein, 9 aa, synthetic construct
GGSGADIIK

SEQ ID NO: 8015 - protein, 9 aa, synthetic construct
GGSGADIFY

SEQ ID NO: 8016 - protein, 9 aa, synthetic construct
GGAGNDVML

SEQ ID NO: 8017 - protein, 9 aa, synthetic construct
GGKGSDKLY

SEQ ID NO: 8018 - protein, 9 aa, synthetic construct
GGAGNDVVN

SEQ ID NO: 8019 - protein, 9 aa, synthetic construct
GGDGDDIIF

SEQ ID NO: 8020 - protein, 9 aa, synthetic construct
GGDGNDSLM

SEQ ID NO: 8021 - protein, 9 aa, synthetic construct
GGKGSDLLT

SEQ ID NO: 8022 - protein, 9 aa, synthetic construct
GGFGTDTLA

SEQ ID NO: 8023 - protein, 9 aa, synthetic construct
GGDGDDLFL

SEQ ID NO: 8024 - protein, 9 aa, synthetic construct
GGDGNDKIN

SEQ ID NO: 8025 - protein, 9 aa, synthetic construct
GGSGADILT

SEQ ID NO: 8026 - protein, 9 aa, synthetic construct
GGDGNDSLR

SEQ ID NO: 8027 - protein, 9 aa, synthetic construct
GGDGDDIFV

SEQ ID NO: 8028 - protein, 9 aa, synthetic construct
GGKGSDTFV

SEQ ID NO: 8029 - protein, 9 aa, synthetic construct
GGRGWDKLW

SEQ ID NO: 8030 - protein, 9 aa, synthetic construct
GGAGNDYFD

SEQ ID NO: 8031 - protein, 9 aa, synthetic construct
GGRGTDTLT

SEQ ID NO: 8032 - protein, 9 aa, synthetic construct
GGKGIDTFT

SEQ ID NO: 8033 - protein, 9 aa, synthetic construct
GGRGTDTIY

SEQ ID NO: 8034 - protein, 9 aa, synthetic construct
GGGGNDQLY

SEQ ID NO: 8035 - protein, 9 aa, synthetic construct
GGKGIDRME

SEQ ID NO: 8036 - protein, 9 aa, synthetic construct
GGKGIDMLY

SEQ ID NO: 8037 - protein, 9 aa, synthetic construct
GGDGNDIVG

SEQ ID NO: 8038 - protein, 9 aa, synthetic construct
GGSGADILE

SEQ ID NO: 8039 - protein, 9 aa, synthetic construct
GGSGADKLN

SEQ ID NO: 8040 - protein, 9 aa, synthetic construct
GGEGHDTYV

SEQ ID NO: 8041 - protein, 9 aa, synthetic construct
GGSGADTFF

SEQ ID NO: 8042 - protein, 9 aa, synthetic construct
GGNGFDILN

SEQ ID NO: 8043 - protein, 9 aa, synthetic construct
GGDGNDSIG

SEQ ID NO: 8044 - protein, 9 aa, synthetic construct
GGSGKDRLT

SEQ ID NO: 8045 - protein, 9 aa, synthetic construct
GGGGNDQLR

SEQ ID NO: 8046 - protein, 9 aa, synthetic construct
GGSGADVMI

SEQ ID NO: 8047 - protein, 9 aa, synthetic construct
GGSGADVIY

SEQ ID NO: 8048 - protein, 9 aa, synthetic construct
GGSGADVII

SEQ ID NO: 8049 - protein, 9 aa, synthetic construct
GGSGADVID

SEQ ID NO: 8050 - protein, 9 aa, synthetic construct
GGSGADVFQ

SEQ ID NO: 8051 - protein, 9 aa, synthetic construct
GGSGKDTFK

SEQ ID NO: 8052 - protein, 9 aa, synthetic construct
GGSGADTIS

SEQ ID NO: 8053 - protein, 9 aa, synthetic construct
GGKGRDRLY

SEQ ID NO: 8054 - protein, 9 aa, synthetic construct
GGSGADTFD

SEQ ID NO: 8055 - protein, 9 aa, synthetic construct
GGNGFDTAS

SEQ ID NO: 8056 - protein, 9 aa, synthetic construct
GGSGADTFA

SEQ ID NO: 8057 - protein, 9 aa, synthetic construct
GGAGNDTME

SEQ ID NO: 8058 - protein, 9 aa, synthetic construct
GGAGNDTVE

SEQ ID NO: 8059 - protein, 9 aa, synthetic construct
GGAGNDTVG

SEQ ID NO: 8060 - protein, 9 aa, synthetic construct
GGAGNDTVK

SEQ ID NO: 8061 - protein, 9 aa, synthetic construct
GGSGADRID

SEQ ID NO: 8062 - protein, 9 aa, synthetic construct
GGDGNDLLH

SEQ ID NO: 8063 - protein, 9 aa, synthetic construct
GGAGNDVFF

SEQ ID NO: 8064 - protein, 9 aa, synthetic construct
GGSGKDVLQ

SEQ ID NO: 8065 - protein, 9 aa, synthetic construct
GGNGFDTAD

SEQ ID NO: 8066 - protein, 9 aa, synthetic construct
GGSGKDVLS

SEQ ID NO: 8067 - protein, 9 aa, synthetic construct
GGSGADLLK

SEQ ID NO: 8068 - protein, 9 aa, synthetic construct
GGEGHDVLS

SEQ ID NO: 8069 - protein, 9 aa, synthetic construct
GGRGSDLVK

SEQ ID NO: 8070 - protein, 9 aa, synthetic construct
GGDGNDFIV

SEQ ID NO: 8071 - protein, 9 aa, synthetic construct
GGLGRDTLI

SEQ ID NO: 8072 - protein, 9 aa, synthetic construct
GGRGNDTYL

SEQ ID NO: 8073 - protein, 9 aa, synthetic construct
GGDGNDSVY

SEQ ID NO: 8074 - protein, 9 aa, synthetic construct
GGLGADKLS

SEQ ID NO: 8075 - protein, 9 aa, synthetic construct
GGRGNDTLH

SEQ ID NO: 8076 - protein, 9 aa, synthetic construct
GGAGNDAMT

SEQ ID NO: 8077 - protein, 9 aa, synthetic construct
GGRGNDTIV

SEQ ID NO: 8078 - protein, 9 aa, synthetic construct
GGAGQDRFV

SEQ ID NO: 8079 - protein, 9 aa, synthetic construct
GGRGNDTIH

SEQ ID NO: 8080 - protein, 9 aa, synthetic construct
GGRGNDTID

SEQ ID NO: 8081 - protein, 9 aa, synthetic construct
GGGGNDKLT

SEQ ID NO: 8082 - protein, 9 aa, synthetic construct
GGLGADLIE

SEQ ID NO: 8083 - protein, 9 aa, synthetic construct
GGLGRDTLN

SEQ ID NO: 8084 - protein, 9 aa, synthetic construct
GGLGRDTLF

SEQ ID NO: 8085 - protein, 9 aa, synthetic construct
GGSGNDALT

SEQ ID NO: 8086 - protein, 9 aa, synthetic construct
GGLGADLLS

SEQ ID NO: 8087 - protein, 9 aa, synthetic construct
GGRGNDRLV

SEQ ID NO: 8088 - protein, 9 aa, synthetic construct
GGRGNDRLN

SEQ ID NO: 8089 - protein, 9 aa, synthetic construct
GGRGNDQLF

SEQ ID NO: 8090 - protein, 9 aa, synthetic construct
GGDGDDFVF

SEQ ID NO: 8091 - protein, 9 aa, synthetic construct
GGAGQDTFQ

SEQ ID NO: 8092 - protein, 9 aa, synthetic construct
GGAGQDTID

SEQ ID NO: 8093 - protein, 9 aa, synthetic construct
GGRGNDLVD

SEQ ID NO: 8094 - protein, 9 aa, synthetic construct
GGRGNDLMD

SEQ ID NO: 8095 - protein, 9 aa, synthetic construct
GGRGNDLLT

SEQ ID NO: 8096 - protein, 9 aa, synthetic construct
GGRGNDLLE

SEQ ID NO: 8097 - protein, 9 aa, synthetic construct
GGLGADNLY

SEQ ID NO: 8098 - protein, 9 aa, synthetic construct
GGRGNDVLE

SEQ ID NO: 8099 - protein, 9 aa, synthetic construct
GGSGNDALR

SEQ ID NO: 8100 - protein, 9 aa, synthetic construct
GGDGNDIIS

SEQ ID NO: 8101 - protein, 9 aa, synthetic construct
GGGGADALY

SEQ ID NO: 8102 - protein, 9 aa, synthetic construct
GGDGNDIIR

SEQ ID NO: 8103 - protein, 9 aa, synthetic construct
GGEGDDTVK

SEQ ID NO: 8104 - protein, 9 aa, synthetic construct
GGRGSDKMT

SEQ ID NO: 8105 - protein, 9 aa, synthetic construct
GGAGPDTFV

SEQ ID NO: 8106 - protein, 9 aa, synthetic construct
GGDGNDIIG

SEQ ID NO: 8107 - protein, 9 aa, synthetic construct
GGDGDDHLW

SEQ ID NO: 8108 - protein, 9 aa, synthetic construct
GGEGHDTLF

SEQ ID NO: 8109 - protein, 9 aa, synthetic construct
GGDGDDHLL

SEQ ID NO: 8110 - protein, 9 aa, synthetic construct
GGDGDDHLI

SEQ ID NO: 8111 - protein, 9 aa, synthetic construct
GGSGMDIAD

SEQ ID NO: 8112 - protein, 9 aa, synthetic construct
GGRGRDSLT

SEQ ID NO: 8113 - protein, 9 aa, synthetic construct
GGGGADALS

SEQ ID NO: 8114 - protein, 9 aa, synthetic construct
GGLGADAMN

SEQ ID NO: 8115 - protein, 9 aa, synthetic construct
GGGGADELY

SEQ ID NO: 8116 - protein, 9 aa, synthetic construct
GGDGDDHIE

SEQ ID NO: 8117 - protein, 9 aa, synthetic construct
GGRGRDHLA

SEQ ID NO: 8118 - protein, 9 aa, synthetic construct
GGLGADDLI

SEQ ID NO: 8119 - protein, 9 aa, synthetic construct
GGDGNDHIS

SEQ ID NO: 8120 - protein, 9 aa, synthetic construct
GGNGGDTLY

SEQ ID NO: 8121 - protein, 9 aa, synthetic construct
GGAGQDKLY

SEQ ID NO: 8122 - protein, 9 aa, synthetic construct
GGAGNDAVY

SEQ ID NO: 8123 - protein, 9 aa, synthetic construct
GGDGNDGLS

SEQ ID NO: 8124 - protein, 9 aa, synthetic construct
GGAGQDLLV

SEQ ID NO: 8125 - protein, 9 aa, synthetic construct
GGDGNDGLA

SEQ ID NO: 8126 - protein, 9 aa, synthetic construct
GGLGADIFK

SEQ ID NO: 8127 - protein, 9 aa, synthetic construct
GGRGNDYLS

SEQ ID NO: 8128 - protein, 9 aa, synthetic construct
GGAGNDTFA

SEQ ID NO: 8129 - protein, 9 aa, synthetic construct
GGEGIDLIF

SEQ ID NO: 8130 - protein, 9 aa, synthetic construct
GGAGNDSYL

SEQ ID NO: 8131 - protein, 9 aa, synthetic construct
GGAGNDQIE

SEQ ID NO: 8132 - protein, 9 aa, synthetic construct
GGAGNDMMF

SEQ ID NO: 8133 - protein, 9 aa, synthetic construct
GGSGEDRLL

SEQ ID NO: 8134 - protein, 9 aa, synthetic construct
GGLGSDILN

SEQ ID NO: 8135 - protein, 9 aa, synthetic construct
GGEGIDTLK

SEQ ID NO: 8136 - protein, 9 aa, synthetic construct
GGAGNDNID

SEQ ID NO: 8137 - protein, 9 aa, synthetic construct
GGAGNDNIL

SEQ ID NO: 8138 - protein, 9 aa, synthetic construct
GGKGNDRLN

SEQ ID NO: 8139 - protein, 9 aa, synthetic construct
GGAGNDNLV

SEQ ID NO: 8140 - protein, 9 aa, synthetic construct
GGSGDDYLN

SEQ ID NO: 8141 - protein, 9 aa, synthetic construct
GGDGNDNLR

SEQ ID NO: 8142 - protein, 9 aa, synthetic construct
GGKGNDTFV

SEQ ID NO: 8143 - protein, 9 aa, synthetic construct
GGKGNDTIK

SEQ ID NO: 8144 - protein, 9 aa, synthetic construct
GGAGNDQIH

SEQ ID NO: 8145 - protein, 9 aa, synthetic construct
GGSGEDTLR

SEQ ID NO: 8146 - protein, 9 aa, synthetic construct
GGSGDDVVD

SEQ ID NO: 8147 - protein, 9 aa, synthetic construct
GGSGDDVLH

SEQ ID NO: 8148 - protein, 9 aa, synthetic construct
GGSGDDVLG

SEQ ID NO: 8149 - protein, 9 aa, synthetic construct
GGSGDDVIN

SEQ ID NO: 8150 - protein, 9 aa, synthetic construct
GGSGDDVIE

SEQ ID NO: 8151 - protein, 9 aa, synthetic construct
GGAGNDQLH

SEQ ID NO: 8152 - protein, 9 aa, synthetic construct
GGAGNDHLA

SEQ ID NO: 8153 - protein, 9 aa, synthetic construct
GGAGNDQLK

SEQ ID NO: 8154 - protein, 9 aa, synthetic construct
GGSGDDTVY

SEQ ID NO: 8155 - protein, 9 aa, synthetic construct
GGDGGDFLL

SEQ ID NO: 8156 - protein, 9 aa, synthetic construct
GGSGDDTIV

SEQ ID NO: 8157 - protein, 9 aa, synthetic construct
GGSGDDTIN

SEQ ID NO: 8158 - protein, 9 aa, synthetic construct
GGLGSDILS

SEQ ID NO: 8159 - protein, 9 aa, synthetic construct
GGSGEDYLE

SEQ ID NO: 8160 - protein, 9 aa, synthetic construct
GGSGDDALN

SEQ ID NO: 8161 - protein, 9 aa, synthetic construct
GGKGNDDYA

SEQ ID NO: 8162 - protein, 9 aa, synthetic construct
GGAGNDIIQ

SEQ ID NO: 8163 - protein, 9 aa, synthetic construct
GGSGHDLIA

SEQ ID NO: 8164 - protein, 9 aa, synthetic construct
GGKGNDFLT

SEQ ID NO: 8165 - protein, 9 aa, synthetic construct
GGKGNDFLV

SEQ ID NO: 8166 - protein, 9 aa, synthetic construct
GGAGNDIYE

SEQ ID NO: 8167 - protein, 9 aa, synthetic construct
GGSGHDAFV

SEQ ID NO: 8168 - protein, 9 aa, synthetic construct
GGDGNDRFF

SEQ ID NO: 8169 - protein, 9 aa, synthetic construct
GGDGNDRIN

SEQ ID NO: 8170 - protein, 9 aa, synthetic construct
GGFGQDVVY

SEQ ID NO: 8171 - protein, 9 aa, synthetic construct
GGAGNDIYQ

SEQ ID NO: 8172 - protein, 9 aa, synthetic construct
GGSGGDTLY

SEQ ID NO: 8173 - protein, 9 aa, synthetic construct
GGSGGDTLD

SEQ ID NO: 8174 - protein, 9 aa, synthetic construct
GGAGNDKMY

SEQ ID NO: 8175 - protein, 9 aa, synthetic construct
GGEGIDVLD

SEQ ID NO: 8176 - protein, 9 aa, synthetic construct
GGAGNDLFD

SEQ ID NO: 8177 - protein, 9 aa, synthetic construct
GGSGHDTLR

SEQ ID NO: 8178 - protein, 9 aa, synthetic construct
GGAGNDLFT

SEQ ID NO: 8179 - protein, 9 aa, synthetic construct
GGAGNDLIK

SEQ ID NO: 8180 - protein, 9 aa, synthetic construct
GGKGNDLIQ

SEQ ID NO: 8181 - protein, 9 aa, synthetic construct
GGAGNDLMA

SEQ ID NO: 8182 - protein, 9 aa, synthetic construct
GGAGNDIAD

SEQ ID NO: 8183 - protein, 9 aa, synthetic construct
GGKGNDLLV

SEQ ID NO: 8184 - protein, 9 aa, synthetic construct
GGAGNDLVE

SEQ ID NO: 8185 - protein, 9 aa, synthetic construct
GGSGHDVLA

SEQ ID NO: 8186 - protein, 9 aa, synthetic construct
GGAGNDLYK

SEQ ID NO: 8187 - protein, 9 aa, synthetic construct
GGSGFDDAH

SEQ ID NO: 8188 - protein, 9 aa, synthetic construct
GGSGDDTFY

SEQ ID NO: 8189 - protein, 9 aa, synthetic construct
GGSGDDTFR

SEQ ID NO: 8190 - protein, 9 aa, synthetic construct
GGFGNDYMD

SEQ ID NO: 8191 - protein, 9 aa, synthetic construct
GGAGNDFLH

SEQ ID NO: 8192 - protein, 9 aa, synthetic construct
GGEGIDQLY

SEQ ID NO: 8193 - protein, 9 aa, synthetic construct
GGAGNDRMV

SEQ ID NO: 8194 - protein, 9 aa, synthetic construct
GGSGDDLMR

SEQ ID NO: 8195 - protein, 9 aa, synthetic construct
GGSGDDLLK

SEQ ID NO: 8196 - protein, 9 aa, synthetic construct
GGSGDDLIY

SEQ ID NO: 8197 - protein, 9 aa, synthetic construct
GGSGDDLIE

SEQ ID NO: 8198 - protein, 9 aa, synthetic construct
GGKGKDTFK

SEQ ID NO: 8199 - protein, 9 aa, synthetic construct
GGKGNDYID

SEQ ID NO: 8200 - protein, 9 aa, synthetic construct
GGAGNDRVY

SEQ ID NO: 8201 - protein, 9 aa, synthetic construct
GGAGNDRYA

SEQ ID NO: 8202 - protein, 9 aa, synthetic construct
GGSGDDKLD

SEQ ID NO: 8203 - protein, 9 aa, synthetic construct
GGKGNDYLR

SEQ ID NO: 8204 - protein, 9 aa, synthetic construct
GGDGNDMLL

SEQ ID NO: 8205 - protein, 9 aa, synthetic construct
GGDGNDRLR

SEQ ID NO: 8206 - protein, 9 aa, synthetic construct
GGSGDDIIF

SEQ ID NO: 8207 - protein, 9 aa, synthetic construct
GGAGNDSFR

SEQ ID NO: 8208 - protein, 9 aa, synthetic construct
GGSGDDHLW

SEQ ID NO: 8209 - protein, 9 aa, synthetic construct
GGSGDDGLF

SEQ ID NO: 8210 - protein, 9 aa, synthetic construct
GGSGDDELY

SEQ ID NO: 8211 - protein, 9 aa, synthetic construct
GGSGDDELR

SEQ ID NO: 8212 - protein, 9 aa, synthetic construct
GGAGNDSMI

SEQ ID NO: 8213 - protein, 9 aa, synthetic construct
GGAGNDFIF

SEQ ID NO: 8214 - protein, 9 aa, synthetic construct
GGGGGDIFD

SEQ ID NO: 8215 - protein, 9 aa, synthetic construct
GGSGDDDLF

SEQ ID NO: 8216 - protein, 9 aa, synthetic construct
GGAGNDSMS

SEQ ID NO: 8217 - protein, 9 aa, synthetic construct
GGDGGDKLY

SEQ ID NO: 8218 - protein, 9 aa, synthetic construct
GGNGDDVLS

SEQ ID NO: 8219 - protein, 9 aa, synthetic construct
GGSGDDMLA

SEQ ID NO: 8220 - protein, 9 aa, synthetic construct
GGKGNDVLW

SEQ ID NO: 8221 - protein, 9 aa, synthetic construct
GGSGIDTLT

SEQ ID NO: 8222 - protein, 9 aa, synthetic construct
GGKGNDTMV

SEQ ID NO: 8223 - protein, 9 aa, synthetic construct
GGSGIDKLT

SEQ ID NO: 8224 - protein, 9 aa, synthetic construct
GGSGDDSYV

SEQ ID NO: 8225 - protein, 9 aa, synthetic construct
GGAGNDQMW

SEQ ID NO: 8226 - protein, 9 aa, synthetic construct
GGDGDDIYI

SEQ ID NO: 8227 - protein, 9 aa, synthetic construct
GGSGDDSVA

SEQ ID NO: 8228 - protein, 9 aa, synthetic construct
GGKGNDTYA

SEQ ID NO: 8229 - protein, 9 aa, synthetic construct
GGKGLDSIV

SEQ ID NO: 8230 - protein, 9 aa, synthetic construct
GGSGDDSLT

SEQ ID NO: 8231 - protein, 9 aa, synthetic construct
GGEGADWLW

SEQ ID NO: 8232 - protein, 9 aa, synthetic construct
GGSGDDRLR

SEQ ID NO: 8233 - protein, 9 aa, synthetic construct
GGSGDDRLG

SEQ ID NO: 8234 - protein, 9 aa, synthetic construct
GGDGNDRMF

SEQ ID NO: 8235 - protein, 9 aa, synthetic construct
GGSGDDRIY

SEQ ID NO: 8236 - protein, 9 aa, synthetic construct
GGGGNDQFR

SEQ ID NO: 8237 - protein, 9 aa, synthetic construct
GGKGNDVLH

SEQ ID NO: 8238 - protein, 9 aa, synthetic construct
GGSGDDRIS

SEQ ID NO: 8239 - protein, 9 aa, synthetic construct
GGFGNDYLD

SEQ ID NO: 8240 - protein, 9 aa, synthetic construct
GGSGDDRIG

SEQ ID NO: 8241 - protein, 9 aa, synthetic construct
GGSGIDTAD

SEQ ID NO: 8242 - protein, 9 aa, synthetic construct
GGKGNDVLL

SEQ ID NO: 8243 - protein, 9 aa, synthetic construct
GGSGDDQLS

SEQ ID NO: 8244 - protein, 9 aa, synthetic construct
GGSGDDQLA

SEQ ID NO: 8245 - protein, 9 aa, synthetic construct
GGDGNDRMY

SEQ ID NO: 8246 - protein, 9 aa, synthetic construct
GGSGIDTLS

SEQ ID NO: 8247 - protein, 9 aa, synthetic construct
GGRGNDILR

SEQ ID NO: 8248 - protein, 9 aa, synthetic construct
GGSGNDELT

SEQ ID NO: 8249 - protein, 9 aa, synthetic construct
GGNGNDALR

SEQ ID NO: 8250 - protein, 9 aa, synthetic construct
GGQGNDLLT

SEQ ID NO: 8251 - protein, 9 aa, synthetic construct
GGAGSDLLA

SEQ ID NO: 8252 - protein, 9 aa, synthetic construct
GGAGSDLLE

SEQ ID NO: 8253 - protein, 9 aa, synthetic construct
GGQGNDSIS

SEQ ID NO: 8254 - protein, 9 aa, synthetic construct
GGKGEDTLR

SEQ ID NO: 8255 - protein, 9 aa, synthetic construct
GGEGDDDLS

SEQ ID NO: 8256 - protein, 9 aa, synthetic construct
GGNGDDTLK

SEQ ID NO: 8257 - protein, 9 aa, synthetic construct
GGQGNDQLF

SEQ ID NO: 8258 - protein, 9 aa, synthetic construct
GGGGADTMA

SEQ ID NO: 8259 - protein, 9 aa, synthetic construct
GGDGNDTMS

SEQ ID NO: 8260 - protein, 9 aa, synthetic construct
GGGGADTML

SEQ ID NO: 8261 - protein, 9 aa, synthetic construct
GGGGADTMT

SEQ ID NO: 8262 - protein, 9 aa, synthetic construct
GGQGNDLMA

SEQ ID NO: 8263 - protein, 9 aa, synthetic construct
GGQGNDLLE

SEQ ID NO: 8264 - protein, 9 aa, synthetic construct
GGAGSDLIY

SEQ ID NO: 8265 - protein, 9 aa, synthetic construct
GGLGDDTIE

SEQ ID NO: 8266 - protein, 9 aa, synthetic construct
GGAGSDMLY

SEQ ID NO: 8267 - protein, 9 aa, synthetic construct
GGLGDDTIT

SEQ ID NO: 8268 - protein, 9 aa, synthetic construct
GGAGSDNLD

SEQ ID NO: 8269 - protein, 9 aa, synthetic construct
GGQGNDFLL

SEQ ID NO: 8270 - protein, 9 aa, synthetic construct
GGQGNDFLI

SEQ ID NO: 8271 - protein, 9 aa, synthetic construct
GGQGNDFLG

SEQ ID NO: 8272 - protein, 9 aa, synthetic construct
GGQGNDFLD

SEQ ID NO: 8273 - protein, 9 aa, synthetic construct
GGAGSDQLS

SEQ ID NO: 8274 - protein, 9 aa, synthetic construct
GGAGSDQLT

SEQ ID NO: 8275 - protein, 9 aa, synthetic construct
GGGGADVFK

SEQ ID NO: 8276 - protein, 9 aa, synthetic construct
GGGGADVFQ

SEQ ID NO: 8277 - protein, 9 aa, synthetic construct
GGSGNDQLS

SEQ ID NO: 8278 - protein, 9 aa, synthetic construct
GGQGNDSLY

SEQ ID NO: 8279 - protein, 9 aa, synthetic construct
GGLGDDVID

SEQ ID NO: 8280 - protein, 9 aa, synthetic construct
GGAGSDILA

SEQ ID NO: 8281 - protein, 9 aa, synthetic construct
GGQGRDVLT

SEQ ID NO: 8282 - protein, 9 aa, synthetic construct
GGDGDDDMM

SEQ ID NO: 8283 - protein, 9 aa, synthetic construct
GGQGRDSLF

SEQ ID NO: 8284 - protein, 9 aa, synthetic construct
GGLGDDQIS

SEQ ID NO: 8285 - protein, 9 aa, synthetic construct
GGGGADTFE

SEQ ID NO: 8286 - protein, 9 aa, synthetic construct
GGQGRDILA

SEQ ID NO: 8287 - protein, 9 aa, synthetic construct
GGEGGDRFV

SEQ ID NO: 8288 - protein, 9 aa, synthetic construct
GGDGDDDLS

SEQ ID NO: 8289 - protein, 9 aa, synthetic construct
GGEGDDDLN

SEQ ID NO: 8290 - protein, 9 aa, synthetic construct
GGQGQDTLS

SEQ ID NO: 8291 - protein, 9 aa, synthetic construct
GGQGQDTLI

SEQ ID NO: 8292 - protein, 9 aa, synthetic construct
GGGGADTFT

SEQ ID NO: 8293 - protein, 9 aa, synthetic construct
GGLGDDRLF

SEQ ID NO: 8294 - protein, 9 aa, synthetic construct
GGAGSDLFN

SEQ ID NO: 8295 - protein, 9 aa, synthetic construct
GGLGDDRLV

SEQ ID NO: 8296 - protein, 9 aa, synthetic construct
GGNGDDTLR

SEQ ID NO: 8297 - protein, 9 aa, synthetic construct
GGQGNDVLN

SEQ ID NO: 8298 - protein, 9 aa, synthetic construct
GGQGNDVLK

SEQ ID NO: 8299 - protein, 9 aa, synthetic construct
GGAGSDKLL

SEQ ID NO: 8300 - protein, 9 aa, synthetic construct
GGGGNDFLN

SEQ ID NO: 8301 - protein, 9 aa, synthetic construct
GGSGNDQIH

SEQ ID NO: 8302 - protein, 9 aa, synthetic construct
GGAGSDKLS

SEQ ID NO: 8303 - protein, 9 aa, synthetic construct
GGLGDDSIE

SEQ ID NO: 8304 - protein, 9 aa, synthetic construct
GGDGDDDLG

SEQ ID NO: 8305 - protein, 9 aa, synthetic construct
GGQGNDTIT

SEQ ID NO: 8306 - protein, 9 aa, synthetic construct
GGQGNDTIE

SEQ ID NO: 8307 - protein, 9 aa, synthetic construct
GGAGSDRIY

SEQ ID NO: 8308 - protein, 9 aa, synthetic construct
GGLGDDVII

SEQ ID NO: 8309 - protein, 9 aa, synthetic construct
GGAGQDTVR

SEQ ID NO: 8310 - protein, 9 aa, synthetic construct
GGSGNDTAT

SEQ ID NO: 8311 - protein, 9 aa, synthetic construct
GGQGDDVIR

SEQ ID NO: 8312 - protein, 9 aa, synthetic construct
GGDGDDALT

SEQ ID NO: 8313 - protein, 9 aa, synthetic construct
GGQGDDTLE

SEQ ID NO: 8314 - protein, 9 aa, synthetic construct
GGSGNDSVD

SEQ ID NO: 8315 - protein, 9 aa, synthetic construct
GGAGSDVLL

SEQ ID NO: 8316 - protein, 9 aa, synthetic construct
GGDGKDVLD

SEQ ID NO: 8317 - protein, 9 aa, synthetic construct
GGGGNDALY

SEQ ID NO: 8318 - protein, 9 aa, synthetic construct
GGLGEDYLL

SEQ ID NO: 8319 - protein, 9 aa, synthetic construct
GGDGKDTLY

SEQ ID NO: 8320 - protein, 9 aa, synthetic construct
GGLGFDLLT

SEQ ID NO: 8321 - protein, 9 aa, synthetic construct
GGQGDDLVY

SEQ ID NO: 8322 - protein, 9 aa, synthetic construct
GGQGDDLLV

SEQ ID NO: 8323 - protein, 9 aa, synthetic construct
GGDGNDTYL

SEQ ID NO: 8324 - protein, 9 aa, synthetic construct
GGQGDDVLA

SEQ ID NO: 8325 - protein, 9 aa, synthetic construct
GGLGFDTLQ

SEQ ID NO: 8326 - protein, 9 aa, synthetic construct
GGAGSDYLR

SEQ ID NO: 8327 - protein, 9 aa, synthetic construct
GGAGSDYLV

SEQ ID NO: 8328 - protein, 9 aa, synthetic construct
GGQGDDIYV

SEQ ID NO: 8329 - protein, 9 aa, synthetic construct
GGSGNDTFY

SEQ ID NO: 8330 - protein, 9 aa, synthetic construct
GGEGDDLLH

SEQ ID NO: 8331 - protein, 9 aa, synthetic construct
GGGGDDALY

SEQ ID NO: 8332 - protein, 9 aa, synthetic construct
GGGGNDAIT

SEQ ID NO: 8333 - protein, 9 aa, synthetic construct
GGNGNDALF

SEQ ID NO: 8334 - protein, 9 aa, synthetic construct
GGDGKDRLK

SEQ ID NO: 8335 - protein, 9 aa, synthetic construct
GGNGNDALM

SEQ ID NO: 8336 - protein, 9 aa, synthetic construct
GGAGTDDLN

SEQ ID NO: 8337 - protein, 9 aa, synthetic construct
GGQGDDVIS

SEQ ID NO: 8338 - protein, 9 aa, synthetic construct
GGQGDDVLS

SEQ ID NO: 8339 - protein, 9 aa, synthetic construct
GGQGKDTYN

SEQ ID NO: 8340 - protein, 9 aa, synthetic construct
GGEGDDLLN

SEQ ID NO: 8341 - protein, 9 aa, synthetic construct
GGAGSDRYV

SEQ ID NO: 8342 - protein, 9 aa, synthetic construct
GGLGDDVLQ

SEQ ID NO: 8343 - protein, 9 aa, synthetic construct
GGSGNDSAS

SEQ ID NO: 8344 - protein, 9 aa, synthetic construct
GGGGADVLF

SEQ ID NO: 8345 - protein, 9 aa, synthetic construct
GGAGSDSIL

SEQ ID NO: 8346 - protein, 9 aa, synthetic construct
GGAGSDSIT

SEQ ID NO: 8347 - protein, 9 aa, synthetic construct
GGAGSDSLA

SEQ ID NO: 8348 - protein, 9 aa, synthetic construct
GGKGDDYLQ

SEQ ID NO: 8349 - protein, 9 aa, synthetic construct
GGNGKDVLI

SEQ ID NO: 8350 - protein, 9 aa, synthetic construct
GGGGNDELD

SEQ ID NO: 8351 - protein, 9 aa, synthetic construct
GGQGGDTLN

SEQ ID NO: 8352 - protein, 9 aa, synthetic construct
GGAGSDTIH

SEQ ID NO: 8353 - protein, 9 aa, synthetic construct
GGKGDDYLD

SEQ ID NO: 8354 - protein, 9 aa, synthetic construct
GGDGKDYLL

SEQ ID NO: 8355 - protein, 9 aa, synthetic construct
GGSGNDSIY

SEQ ID NO: 8356 - protein, 9 aa, synthetic construct
GGAGSDTIL

SEQ ID NO: 8357 - protein, 9 aa, synthetic construct
GGQGFDVID

SEQ ID NO: 8358 - protein, 9 aa, synthetic construct
GGEGDDELH

SEQ ID NO: 8359 - protein, 9 aa, synthetic construct
GGDGGDTLL

SEQ ID NO: 8360 - protein, 9 aa, synthetic construct
GGQGEDRLD

SEQ ID NO: 8361 - protein, 9 aa, synthetic construct
GGNGLDNFI

SEQ ID NO: 8362 - protein, 9 aa, synthetic construct
GGGGNDDLS

SEQ ID NO: 8363 - protein, 9 aa, synthetic construct
GGLGEDILT

SEQ ID NO: 8364 - protein, 9 aa, synthetic construct
GGEGGDFLL

SEQ ID NO: 8365 - protein, 9 aa, synthetic construct
GGGGADWLS

SEQ ID NO: 8366 - protein, 9 aa, synthetic construct
GGQGDDWLE

SEQ ID NO: 8367 - protein, 9 aa, synthetic construct
GGAGSDFAL

SEQ ID NO: 8368 - protein, 9 aa, synthetic construct
GGSGNDMLS

SEQ ID NO: 8369 - protein, 9 aa, synthetic construct
GGSGNDMLN

SEQ ID NO: 8370 - protein, 9 aa, synthetic construct
GGSGNDIIS

SEQ ID NO: 8371 - protein, 9 aa, synthetic construct
GGRGDDVLA

SEQ ID NO: 8372 - protein, 9 aa, synthetic construct
GGAGRDLLY

SEQ ID NO: 8373 - protein, 9 aa, synthetic construct
GGNGDDTMY

SEQ ID NO: 8374 - protein, 9 aa, synthetic construct
GGRGDDTAL

SEQ ID NO: 8375 - protein, 9 aa, synthetic construct
GGLGADVMY

SEQ ID NO: 8376 - protein, 9 aa, synthetic construct
GGRGDDSLK

SEQ ID NO: 8377 - protein, 9 aa, synthetic construct
GGRGDDSLF

SEQ ID NO: 8378 - protein, 9 aa, synthetic construct
GGAGRDMLF

SEQ ID NO: 8379 - protein, 9 aa, synthetic construct
GGAGRDMLS

SEQ ID NO: 8380 - protein, 9 aa, synthetic construct
GGRGDDRLT

SEQ ID NO: 8381 - protein, 9 aa, synthetic construct
GGRGDDRIQ

SEQ ID NO: 8382 - protein, 9 aa, synthetic construct
GGDGNDDLD

SEQ ID NO: 8383 - protein, 9 aa, synthetic construct
GGNGHDVLI

SEQ ID NO: 8384 - protein, 9 aa, synthetic construct
GGAGRDLLF

SEQ ID NO: 8385 - protein, 9 aa, synthetic construct
GGLGRDRLE

SEQ ID NO: 8386 - protein, 9 aa, synthetic construct
GGLGDDAFV

SEQ ID NO: 8387 - protein, 9 aa, synthetic construct
GGGGNDILE

SEQ ID NO: 8388 - protein, 9 aa, synthetic construct
GGRGDDLVS

SEQ ID NO: 8389 - protein, 9 aa, synthetic construct
GGSGNDILH

SEQ ID NO: 8390 - protein, 9 aa, synthetic construct
GGRGDDLLV

SEQ ID NO: 8391 - protein, 9 aa, synthetic construct
GGRGDDLLS

SEQ ID NO: 8392 - protein, 9 aa, synthetic construct
GGRGDDLLL

SEQ ID NO: 8393 - protein, 9 aa, synthetic construct
GGLGDDAMY

SEQ ID NO: 8394 - protein, 9 aa, synthetic construct
GGSGNDILQ

SEQ ID NO: 8395 - protein, 9 aa, synthetic construct
GGRGDDLIS

SEQ ID NO: 8396 - protein, 9 aa, synthetic construct
GGRGDDLIR

SEQ ID NO: 8397 - protein, 9 aa, synthetic construct
GGRGDDVLR

SEQ ID NO: 8398 - protein, 9 aa, synthetic construct
GGNGHDTLN

SEQ ID NO: 8399 - protein, 9 aa, synthetic construct
GGGGADSLE

SEQ ID NO: 8400 - protein, 9 aa, synthetic construct
GGAGRDELS

SEQ ID NO: 8401 - protein, 9 aa, synthetic construct
GGAGQDVFE

SEQ ID NO: 8402 - protein, 9 aa, synthetic construct
GGAGNDAIH

SEQ ID NO: 8403 - protein, 9 aa, synthetic construct
GGRGNDELD

SEQ ID NO: 8404 - protein, 9 aa, synthetic construct
GGGGADIFR

SEQ ID NO: 8405 - protein, 9 aa, synthetic construct
GGGGADIFS

SEQ ID NO: 8406 - protein, 9 aa, synthetic construct
GGGGADIIT

SEQ ID NO: 8407 - protein, 9 aa, synthetic construct
GGAGRDALN

SEQ ID NO: 8408 - protein, 9 aa, synthetic construct
GGLGADRMV

SEQ ID NO: 8409 - protein, 9 aa, synthetic construct
GGGGNDIYY

SEQ ID NO: 8410 - protein, 9 aa, synthetic construct
GGDGNDEMD

SEQ ID NO: 8411 - protein, 9 aa, synthetic construct
GGRGKDKLT

SEQ ID NO: 8412 - protein, 9 aa, synthetic construct
GGDGNDELR

SEQ ID NO: 8413 - protein, 9 aa, synthetic construct
GGDGGDRLD

SEQ ID NO: 8414 - protein, 9 aa, synthetic construct
GGGGADLLR

SEQ ID NO: 8415 - protein, 9 aa, synthetic construct
GGRGGDVMW

SEQ ID NO: 8416 - protein, 9 aa, synthetic construct
GGFGNDTIH

SEQ ID NO: 8417 - protein, 9 aa, synthetic construct
GGLGADTLQ

SEQ ID NO: 8418 - protein, 9 aa, synthetic construct
GGLGADTML

SEQ ID NO: 8419 - protein, 9 aa, synthetic construct
GGAGMDVMS

SEQ ID NO: 8420 - protein, 9 aa, synthetic construct
GGRGGDALF

SEQ ID NO: 8421 - protein, 9 aa, synthetic construct
GGFGNDTID

SEQ ID NO: 8422 - protein, 9 aa, synthetic construct
GGRGFDHLF

SEQ ID NO: 8423 - protein, 9 aa, synthetic construct
GGGGADLIR

SEQ ID NO: 8424 - protein, 9 aa, synthetic construct
GGAGRDKLI

SEQ ID NO: 8425 - protein, 9 aa, synthetic construct
GGSGNDGIS

SEQ ID NO: 8426 - protein, 9 aa, synthetic construct
GGLGADVFR

SEQ ID NO: 8427 - protein, 9 aa, synthetic construct
GGLGDDDLD

SEQ ID NO: 8428 - protein, 9 aa, synthetic construct
GGLGDDDLT

SEQ ID NO: 8429 - protein, 9 aa, synthetic construct
GGSGNDIML

SEQ ID NO: 8430 - protein, 9 aa, synthetic construct
GGGGADRMA

SEQ ID NO: 8431 - protein, 9 aa, synthetic construct
GGAGRDVFR

SEQ ID NO: 8432 - protein, 9 aa, synthetic construct
GGAGRDVID

SEQ ID NO: 8433 - protein, 9 aa, synthetic construct
GGLGRDMLT

SEQ ID NO: 8434 - protein, 9 aa, synthetic construct
GGAGRDVMQ

SEQ ID NO: 8435 - protein, 9 aa, synthetic construct
GGDGMDSFV

SEQ ID NO: 8436 - protein, 9 aa, synthetic construct
GGLGDDKLS

SEQ ID NO: 8437 - protein, 9 aa, synthetic construct
GGLGDDKLW

SEQ ID NO: 8438 - protein, 9 aa, synthetic construct
GGLGDDKLY

SEQ ID NO: 8439 - protein, 9 aa, synthetic construct
GGGGADRIY

SEQ ID NO: 8440 - protein, 9 aa, synthetic construct
GGSGNDLME

SEQ ID NO: 8441 - protein, 9 aa, synthetic construct
GGLGDDLIL

SEQ ID NO: 8442 - protein, 9 aa, synthetic construct
GGAGRDYLS

SEQ ID NO: 8443 - protein, 9 aa, synthetic construct
GGAGSDALR

SEQ ID NO: 8444 - protein, 9 aa, synthetic construct
GGLGDDDVF

SEQ ID NO: 8445 - protein, 9 aa, synthetic construct
GGAGSDALY

SEQ ID NO: 8446 - protein, 9 aa, synthetic construct
GGLGDDLLQ

SEQ ID NO: 8447 - protein, 9 aa, synthetic construct
GGEGDDDIL

SEQ ID NO: 8448 - protein, 9 aa, synthetic construct
GGAGSDDLF

SEQ ID NO: 8449 - protein, 9 aa, synthetic construct
GGAGMDQLA

SEQ ID NO: 8450 - protein, 9 aa, synthetic construct
GGFGNDRLY

SEQ ID NO: 8451 - protein, 9 aa, synthetic construct
GGEGDDVIG

SEQ ID NO: 8452 - protein, 9 aa, synthetic construct
GGNGIDVLN

SEQ ID NO: 8453 - protein, 9 aa, synthetic construct
GGLGRDLLI

SEQ ID NO: 8454 - protein, 9 aa, synthetic construct
GGGGNDGLN

SEQ ID NO: 8455 - protein, 9 aa, synthetic construct
GGFGNDRLH

SEQ ID NO: 8456 - protein, 9 aa, synthetic construct
GGGGADSLA

SEQ ID NO: 8457 - protein, 9 aa, synthetic construct
GGRGADHLN

SEQ ID NO: 8458 - protein, 9 aa, synthetic construct
GGSGNDLIV

SEQ ID NO: 8459 - protein, 9 aa, synthetic construct
GGRGADKLW

SEQ ID NO: 8460 - protein, 9 aa, synthetic construct
GGRGADLFV

SEQ ID NO: 8461 - protein, 9 aa, synthetic construct
GGDGDDEMH

SEQ ID NO: 8462 - protein, 9 aa, synthetic construct
GGAGRDSFL

SEQ ID NO: 8463 - protein, 9 aa, synthetic construct
GGAGRDSLF

SEQ ID NO: 8464 - protein, 9 aa, synthetic construct
GGAGRDSLI

SEQ ID NO: 8465 - protein, 9 aa, synthetic construct
GGSGNDKID

SEQ ID NO: 8466 - protein, 9 aa, synthetic construct
GGDGNDAIT

SEQ ID NO: 8467 - protein, 9 aa, synthetic construct
GGLGDDFLD

SEQ ID NO: 8468 - protein, 9 aa, synthetic construct
GGGGADQFV

SEQ ID NO: 8469 - protein, 9 aa, synthetic construct
GGLGDDFMV

SEQ ID NO: 8470 - protein, 9 aa, synthetic construct
GGNGIDKID

SEQ ID NO: 8471 - protein, 9 aa, synthetic construct
GGEGKDSYD

SEQ ID NO: 8472 - protein, 9 aa, synthetic construct
GGRGADTMR

SEQ ID NO: 8473 - protein, 9 aa, synthetic construct
GGRGADTME

SEQ ID NO: 8474 - protein, 9 aa, synthetic construct
GGRGADTLE

SEQ ID NO: 8475 - protein, 9 aa, synthetic construct
GGAGRDTIE

SEQ ID NO: 8476 - protein, 9 aa, synthetic construct
GGGGNDIFV

SEQ ID NO: 8477 - protein, 9 aa, synthetic construct
GGRGADSLS

SEQ ID NO: 8478 - protein, 9 aa, synthetic construct
GGAGRDTLK

SEQ ID NO: 8479 - protein, 9 aa, synthetic construct
GGFGNDSID

SEQ ID NO: 8480 - protein, 9 aa, synthetic construct
GGSGNDKMS

SEQ ID NO: 8481 - protein, 9 aa, synthetic construct
GGRGADRLH

SEQ ID NO: 8482 - protein, 9 aa, synthetic construct
GGRGADRLD

SEQ ID NO: 8483 - protein, 9 aa, synthetic construct
GGSGNDLIF

SEQ ID NO: 8484 - protein, 9 aa, synthetic construct
GGDGDDEIV

SEQ ID NO: 8485 - protein, 9 aa, synthetic construct
GGLGDDILF

SEQ ID NO: 8486 - protein, 9 aa, synthetic construct
GGFGNDQLW

SEQ ID NO: 8487 - protein, 9 aa, synthetic construct
GGGGIDYAL

SEQ ID NO: 8488 - protein, 9 aa, synthetic construct
GGEGDDSLT

SEQ ID NO: 8489 - protein, 9 aa, synthetic construct
GGEGDDTIN

SEQ ID NO: 8490 - protein, 9 aa, synthetic construct
GGVGADLLN

SEQ ID NO: 8491 - protein, 9 aa, synthetic construct
GGAGIDTAL

SEQ ID NO: 8492 - protein, 9 aa, synthetic construct
GGAGDDQVG

SEQ ID NO: 8493 - protein, 9 aa, synthetic construct
GGDGDDVFD

SEQ ID NO: 8494 - protein, 9 aa, synthetic construct
GGKGADDFV

SEQ ID NO: 8495 - protein, 9 aa, synthetic construct
GGKGADALY

SEQ ID NO: 8496 - protein, 9 aa, synthetic construct
GGVGADILI

SEQ ID NO: 8497 - protein, 9 aa, synthetic construct
GGEGNDIIF

SEQ ID NO: 8498 - protein, 9 aa, synthetic construct
GGVGADDLT

SEQ ID NO: 8499 - protein, 9 aa, synthetic construct
GGAGDDRIN

SEQ ID NO: 8500 - protein, 9 aa, synthetic construct
GGHGWDQLY

SEQ ID NO: 8501 - protein, 9 aa, synthetic construct
GGAGDDRLM

SEQ ID NO: 8502 - protein, 9 aa, synthetic construct
GGIGADDMD

SEQ ID NO: 8503 - protein, 9 aa, synthetic construct
GGAGDDTAL

SEQ ID NO: 8504 - protein, 9 aa, synthetic construct
GGDGDDTYH

SEQ ID NO: 8505 - protein, 9 aa, synthetic construct
GGDGSDVLV

SEQ ID NO: 8506 - protein, 9 aa, synthetic construct
GGTGVDVMD

SEQ ID NO: 8507 - protein, 9 aa, synthetic construct
GGTGVDTMT

SEQ ID NO: 8508 - protein, 9 aa, synthetic construct
GGTGVDTLK

SEQ ID NO: 8509 - protein, 9 aa, synthetic construct
GGTGVDTLF

SEQ ID NO: 8510 - protein, 9 aa, synthetic construct
GGAGDDSIN

SEQ ID NO: 8511 - protein, 9 aa, synthetic construct
GGMGSDTLF

SEQ ID NO: 8512 - protein, 9 aa, synthetic construct
GGEGNDFID

SEQ ID NO: 8513 - protein, 9 aa, synthetic construct
GGTGVDIID

SEQ ID NO: 8514 - protein, 9 aa, synthetic construct
GGAGIDSLF

SEQ ID NO: 8515 - protein, 9 aa, synthetic construct
GGEGNDFIG

SEQ ID NO: 8516 - protein, 9 aa, synthetic construct
GGDGFDIAS

SEQ ID NO: 8517 - protein, 9 aa, synthetic construct
GGAGDDQLQ

SEQ ID NO: 8518 - protein, 9 aa, synthetic construct
GGAGDDQLI

SEQ ID NO: 8519 - protein, 9 aa, synthetic construct
GGSGVDVAR

SEQ ID NO: 8520 - protein, 9 aa, synthetic construct
GGSGVDRLY

SEQ ID NO: 8521 - protein, 9 aa, synthetic construct
GGEGSDRLS

SEQ ID NO: 8522 - protein, 9 aa, synthetic construct
GGAGDDMLM

SEQ ID NO: 8523 - protein, 9 aa, synthetic construct
GGAGDDMLN

SEQ ID NO: 8524 - protein, 9 aa, synthetic construct
GGAGDDMLT

SEQ ID NO: 8525 - protein, 9 aa, synthetic construct
GGEGADQLN

SEQ ID NO: 8526 - protein, 9 aa, synthetic construct
GGAGDDNLL

SEQ ID NO: 8527 - protein, 9 aa, synthetic construct
GGDGDDVIM

SEQ ID NO: 8528 - protein, 9 aa, synthetic construct
GGHGRDGLV

SEQ ID NO: 8529 - protein, 9 aa, synthetic construct
GGKGADELI

SEQ ID NO: 8530 - protein, 9 aa, synthetic construct
GGFGDDVLI

SEQ ID NO: 8531 - protein, 9 aa, synthetic construct
GGVGADVLN

SEQ ID NO: 8532 - protein, 9 aa, synthetic construct
GGVGADVLL

SEQ ID NO: 8533 - protein, 9 aa, synthetic construct
GGAGIDTID

SEQ ID NO: 8534 - protein, 9 aa, synthetic construct
GGGGRDILI

SEQ ID NO: 8535 - protein, 9 aa, synthetic construct
GGVGADTMT

SEQ ID NO: 8536 - protein, 9 aa, synthetic construct
GGSGVDTLY

SEQ ID NO: 8537 - protein, 9 aa, synthetic construct
GGVGADTLL

SEQ ID NO: 8538 - protein, 9 aa, synthetic construct
GGVGADTLE

SEQ ID NO: 8539 - protein, 9 aa, synthetic construct
GGVGADTIS

SEQ ID NO: 8540 - protein, 9 aa, synthetic construct
GGVGADSLS

SEQ ID NO: 8541 - protein, 9 aa, synthetic construct
GGVGADSLD

SEQ ID NO: 8542 - protein, 9 aa, synthetic construct
GGVGADRLY

SEQ ID NO: 8543 - protein, 9 aa, synthetic construct
GGVGADQLN

SEQ ID NO: 8544 - protein, 9 aa, synthetic construct
GGAGIDTAY

SEQ ID NO: 8545 - protein, 9 aa, synthetic construct
GGMGSDTYV

SEQ ID NO: 8546 - protein, 9 aa, synthetic construct
GGGGHDRLN

SEQ ID NO: 8547 - protein, 9 aa, synthetic construct
GGKGADFID

SEQ ID NO: 8548 - protein, 9 aa, synthetic construct
GGIGADSLT

SEQ ID NO: 8549 - protein, 9 aa, synthetic construct
GGAGDDVFR

SEQ ID NO: 8550 - protein, 9 aa, synthetic construct
GGAGDDVIK

SEQ ID NO: 8551 - protein, 9 aa, synthetic construct
GGTGSDTLA

SEQ ID NO: 8552 - protein, 9 aa, synthetic construct
GGTGSDTIT

SEQ ID NO: 8553 - protein, 9 aa, synthetic construct
GGGGNDTFL

SEQ ID NO: 8554 - protein, 9 aa, synthetic construct
GGTGSDTIM

SEQ ID NO: 8555 - protein, 9 aa, synthetic construct
GGTGSDTFR

SEQ ID NO: 8556 - protein, 9 aa, synthetic construct
GGEGADRLV

SEQ ID NO: 8557 - protein, 9 aa, synthetic construct
GGTGSDSVS

SEQ ID NO: 8558 - protein, 9 aa, synthetic construct
GGTGADAMA

SEQ ID NO: 8559 - protein, 9 aa, synthetic construct
GGAGDDVLG

SEQ ID NO: 8560 - protein, 9 aa, synthetic construct
GGTGSDSLI

SEQ ID NO: 8561 - protein, 9 aa, synthetic construct
GGIGADSMT

SEQ ID NO: 8562 - protein, 9 aa, synthetic construct
GGTGTDVFL

SEQ ID NO: 8563 - protein, 9 aa, synthetic construct
GGTGSDRIQ

SEQ ID NO: 8564 - protein, 9 aa, synthetic construct
GGTGSDRFV

SEQ ID NO: 8565 - protein, 9 aa, synthetic construct
GGDGSDTIS

SEQ ID NO: 8566 - protein, 9 aa, synthetic construct
GGAGDDVMN

SEQ ID NO: 8567 - protein, 9 aa, synthetic construct
GGAGDDVVD

SEQ ID NO: 8568 - protein, 9 aa, synthetic construct
GGLGTDTLA

SEQ ID NO: 8569 - protein, 9 aa, synthetic construct
GGDGSDTIN

SEQ ID NO: 8570 - protein, 9 aa, synthetic construct
GGAGDDVYF

SEQ ID NO: 8571 - protein, 9 aa, synthetic construct
GGAGDDVYR

SEQ ID NO: 8572 - protein, 9 aa, synthetic construct
GGTGADDMA

SEQ ID NO: 8573 - protein, 9 aa, synthetic construct
GGEGSDVLD

SEQ ID NO: 8574 - protein, 9 aa, synthetic construct
GGNGADEIH

SEQ ID NO: 8575 - protein, 9 aa, synthetic construct
GGTGSDVFV

SEQ ID NO: 8576 - protein, 9 aa, synthetic construct
GGTGSDVIE

SEQ ID NO: 8577 - protein, 9 aa, synthetic construct
GGTGSDVLS

SEQ ID NO: 8578 - protein, 9 aa, synthetic construct
GGSGYDVLI

SEQ ID NO: 8579 - protein, 9 aa, synthetic construct
GGAGDDTFA

SEQ ID NO: 8580 - protein, 9 aa, synthetic construct
GGFGDDTVN

SEQ ID NO: 8581 - protein, 9 aa, synthetic construct
GGTGTDTLY

SEQ ID NO: 8582 - protein, 9 aa, synthetic construct
GGTGTDTLV

SEQ ID NO: 8583 - protein, 9 aa, synthetic construct
GGTGTDTLA

SEQ ID NO: 8584 - protein, 9 aa, synthetic construct
GGAGDDTFT

SEQ ID NO: 8585 - protein, 9 aa, synthetic construct
GGTGTDTFV

SEQ ID NO: 8586 - protein, 9 aa, synthetic construct
GGDGSDTYR

SEQ ID NO: 8587 - protein, 9 aa, synthetic construct
GGAGDDTIM

SEQ ID NO: 8588 - protein, 9 aa, synthetic construct
GGTGTDRLS

SEQ ID NO: 8589 - protein, 9 aa, synthetic construct
GGTGTDRLD

SEQ ID NO: 8590 - protein, 9 aa, synthetic construct
GGAGDDTMA

SEQ ID NO: 8591 - protein, 9 aa, synthetic construct
GGTGTDNLI

SEQ ID NO: 8592 - protein, 9 aa, synthetic construct
GGAGDDTMF

SEQ ID NO: 8593 - protein, 9 aa, synthetic construct
GGDGDDTMT

SEQ ID NO: 8594 - protein, 9 aa, synthetic construct
GGTGTDLLD

SEQ ID NO: 8595 - protein, 9 aa, synthetic construct
GGDGDDTMM

SEQ ID NO: 8596 - protein, 9 aa, synthetic construct
GGIGADRFV

SEQ ID NO: 8597 - protein, 9 aa, synthetic construct
GGIGADRLD

SEQ ID NO: 8598 - protein, 9 aa, synthetic construct
GGSGYDTLR

SEQ ID NO: 8599 - protein, 9 aa, synthetic construct
GGSGYDTLS

SEQ ID NO: 8600 - protein, 9 aa, synthetic construct
GGTGSDYLD

SEQ ID NO: 8601 - protein, 9 aa, synthetic construct
GGFGDDTLY

SEQ ID NO: 8602 - protein, 9 aa, synthetic construct
GGIGADRME

SEQ ID NO: 8603 - protein, 9 aa, synthetic construct
GGEGADRLS

SEQ ID NO: 8604 - protein, 9 aa, synthetic construct
GGVGDDILD

SEQ ID NO: 8605 - protein, 9 aa, synthetic construct
GGVGDDIMR

SEQ ID NO: 8606 - protein, 9 aa, synthetic construct
GGIGADVLN

SEQ ID NO: 8607 - protein, 9 aa, synthetic construct
GGAGDDEIT

SEQ ID NO: 8608 - protein, 9 aa, synthetic construct
GGEGNDVLQ

SEQ ID NO: 8609 - protein, 9 aa, synthetic construct
GGEGSDDLS

SEQ ID NO: 8610 - protein, 9 aa, synthetic construct
GGKGADRLI

SEQ ID NO: 8611 - protein, 9 aa, synthetic construct
GGHGDDRLE

SEQ ID NO: 8612 - protein, 9 aa, synthetic construct
GGVGNDTYY

SEQ ID NO: 8613 - protein, 9 aa, synthetic construct
GGVGNDTYK

SEQ ID NO: 8614 - protein, 9 aa, synthetic construct
GGEGSDELN

SEQ ID NO: 8615 - protein, 9 aa, synthetic construct
GGVGNDSLL

SEQ ID NO: 8616 - protein, 9 aa, synthetic construct
GGVGNDSID

SEQ ID NO: 8617 - protein, 9 aa, synthetic construct
GGEGNDVLA

SEQ ID NO: 8618 - protein, 9 aa, synthetic construct
GGAGDDEIR

SEQ ID NO: 8619 - protein, 9 aa, synthetic construct
GGKGADRFV

SEQ ID NO: 8620 - protein, 9 aa, synthetic construct
GGAGDDEIY

SEQ ID NO: 8621 - protein, 9 aa, synthetic construct
GGGGNDSIE

SEQ ID NO: 8622 - protein, 9 aa, synthetic construct
GGVGNDRLV

SEQ ID NO: 8623 - protein, 9 aa, synthetic construct
GGAGKDGMF

SEQ ID NO: 8624 - protein, 9 aa, synthetic construct
GGHGDDTVI

SEQ ID NO: 8625 - protein, 9 aa, synthetic construct
GGEGNDVIT

SEQ ID NO: 8626 - protein, 9 aa, synthetic construct
GGKGADQLL

SEQ ID NO: 8627 - protein, 9 aa, synthetic construct
GGAGDDEVD

SEQ ID NO: 8628 - protein, 9 aa, synthetic construct
GGKGADQLF

SEQ ID NO: 8629 - protein, 9 aa, synthetic construct
GGDGDDWLA

SEQ ID NO: 8630 - protein, 9 aa, synthetic construct
GGAGDDEVR

SEQ ID NO: 8631 - protein, 9 aa, synthetic construct
GGEGNDVID

SEQ ID NO: 8632 - protein, 9 aa, synthetic construct
GGVGNDMIW

SEQ ID NO: 8633 - protein, 9 aa, synthetic construct
GGVGNDLLS

SEQ ID NO: 8634 - protein, 9 aa, synthetic construct
GGAGDDAYV

SEQ ID NO: 8635 - protein, 9 aa, synthetic construct
GGDGNDYYY

SEQ ID NO: 8636 - protein, 9 aa, synthetic construct
GGSGSDVIY

SEQ ID NO: 8637 - protein, 9 aa, synthetic construct
GGVGRDTFV

SEQ ID NO: 8638 - protein, 9 aa, synthetic construct
GGAGADVMF

SEQ ID NO: 8639 - protein, 9 aa, synthetic construct
GGSGSDSLF

SEQ ID NO: 8640 - protein, 9 aa, synthetic construct
GGAGADVMR

SEQ ID NO: 8641 - protein, 9 aa, synthetic construct
GGEGADLLE

SEQ ID NO: 8642 - protein, 9 aa, synthetic construct
GGAGADVYL

SEQ ID NO: 8643 - protein, 9 aa, synthetic construct
GGLGVDTLK

SEQ ID NO: 8644 - protein, 9 aa, synthetic construct
GGEGADLLI

SEQ ID NO: 8645 - protein, 9 aa, synthetic construct
GGEGADLLK

SEQ ID NO: 8646 - protein, 9 aa, synthetic construct
GGAGADWIF

SEQ ID NO: 8647 - protein, 9 aa, synthetic construct
GGSGSDTIY

SEQ ID NO: 8648 - protein, 9 aa, synthetic construct
GGEGRDTYD

SEQ ID NO: 8649 - protein, 9 aa, synthetic construct
GGSGSDTLK

SEQ ID NO: 8650 - protein, 9 aa, synthetic construct
GGEGRDTYV

SEQ ID NO: 8651 - protein, 9 aa, synthetic construct
GGEGNDVVR

SEQ ID NO: 8652 - protein, 9 aa, synthetic construct
GGAGADWMS

SEQ ID NO: 8653 - protein, 9 aa, synthetic construct
GGVGSDILT

SEQ ID NO: 8654 - protein, 9 aa, synthetic construct
GGGGRDTLR

SEQ ID NO: 8655 - protein, 9 aa, synthetic construct
GGEGNDVVL

SEQ ID NO: 8656 - protein, 9 aa, synthetic construct
GGAGADYID

SEQ ID NO: 8657 - protein, 9 aa, synthetic construct
GGAGADYLT

SEQ ID NO: 8658 - protein, 9 aa, synthetic construct
GGSGSDVFA

SEQ ID NO: 8659 - protein, 9 aa, synthetic construct
GGSGSDVFI

SEQ ID NO: 8660 - protein, 9 aa, synthetic construct
GGVGRDTLT

SEQ ID NO: 8661 - protein, 9 aa, synthetic construct
GGVGRDTLS

SEQ ID NO: 8662 - protein, 9 aa, synthetic construct
GGVGRDTLL

SEQ ID NO: 8663 - protein, 9 aa, synthetic construct
GGVGNDLLF

SEQ ID NO: 8664 - protein, 9 aa, synthetic construct
GGVGNDIYV

SEQ ID NO: 8665 - protein, 9 aa, synthetic construct
GGSGVDQLF

SEQ ID NO: 8666 - protein, 9 aa, synthetic construct
GGVGDDVLA

SEQ ID NO: 8667 - protein, 9 aa, synthetic construct
GGAGDDIYA

SEQ ID NO: 8668 - protein, 9 aa, synthetic construct
GGSGTDWFV

SEQ ID NO: 8669 - protein, 9 aa, synthetic construct
GGDGTDRLY

SEQ ID NO: 8670 - protein, 9 aa, synthetic construct
GGLGVDILR

SEQ ID NO: 8671 - protein, 9 aa, synthetic construct
GGLGVDILK

SEQ ID NO: 8672 - protein, 9 aa, synthetic construct
GGEGNDTMV

SEQ ID NO: 8673 - protein, 9 aa, synthetic construct
GGAGDDKLN

SEQ ID NO: 8674 - protein, 9 aa, synthetic construct
GGAGDDKLV

SEQ ID NO: 8675 - protein, 9 aa, synthetic construct
GGGGNDSLK

SEQ ID NO: 8676 - protein, 9 aa, synthetic construct
GGVGDDVLV

SEQ ID NO: 8677 - protein, 9 aa, synthetic construct
GGVGDDVLN

SEQ ID NO: 8678 - protein, 9 aa, synthetic construct
GGVGDDVLH

SEQ ID NO: 8679 - protein, 9 aa, synthetic construct
GGVGDDTYH

SEQ ID NO: 8680 - protein, 9 aa, synthetic construct
GGAGDDFLG

SEQ ID NO: 8681 - protein, 9 aa, synthetic construct
GGHGNDTIF

SEQ ID NO: 8682 - protein, 9 aa, synthetic construct
GGVGDDTLQ

SEQ ID NO: 8683 - protein, 9 aa, synthetic construct
GGVGDDTLF

SEQ ID NO: 8684 - protein, 9 aa, synthetic construct
GGAGDDLIN

SEQ ID NO: 8685 - protein, 9 aa, synthetic construct
GGVGDDSLD

SEQ ID NO: 8686 - protein, 9 aa, synthetic construct
GGAGDDLMA

SEQ ID NO: 8687 - protein, 9 aa, synthetic construct
GGAGDDLMT

SEQ ID NO: 8688 - protein, 9 aa, synthetic construct
GGAGIDTVT

SEQ ID NO: 8689 - protein, 9 aa, synthetic construct
GGGGNDSLR

SEQ ID NO: 8690 - protein, 9 aa, synthetic construct
GGVGDDLLV

SEQ ID NO: 8691 - protein, 9 aa, synthetic construct
GGAGDDLYR

SEQ ID NO: 8692 - protein, 9 aa, synthetic construct
GGDGQDALF

SEQ ID NO: 8693 - protein, 9 aa, synthetic construct
GGVGGDTLS

SEQ ID NO: 8694 - protein, 9 aa, synthetic construct
GGSGTDVLY

SEQ ID NO: 8695 - protein, 9 aa, synthetic construct
GGEGSDLLN

SEQ ID NO: 8696 - protein, 9 aa, synthetic construct
GGAGKDAID

SEQ ID NO: 8697 - protein, 9 aa, synthetic construct
GGVGNDFLH

SEQ ID NO: 8698 - protein, 9 aa, synthetic construct
GGDGDDVVS

SEQ ID NO: 8699 - protein, 9 aa, synthetic construct
GGSGTDSLV

SEQ ID NO: 8700 - protein, 9 aa, synthetic construct
GGDGTDTLV

SEQ ID NO: 8701 - protein, 9 aa, synthetic construct
GGAGDDGLR

SEQ ID NO: 8702 - protein, 9 aa, synthetic construct
GGAGDDGLT

SEQ ID NO: 8703 - protein, 9 aa, synthetic construct
GGDGTDTLL

SEQ ID NO: 8704 - protein, 9 aa, synthetic construct
GGEGSDILV

SEQ ID NO: 8705 - protein, 9 aa, synthetic construct
GGDGTDTIS

SEQ ID NO: 8706 - protein, 9 aa, synthetic construct
GGAGDDHLF

SEQ ID NO: 8707 - protein, 9 aa, synthetic construct
GGAGKDALT

SEQ ID NO: 8708 - protein, 9 aa, synthetic construct
GGDGDDMLD

SEQ ID NO: 8709 - protein, 9 aa, synthetic construct
GGVGKDTLL

SEQ ID NO: 8710 - protein, 9 aa, synthetic construct
GGDGFDELK

SEQ ID NO: 8711 - protein, 9 aa, synthetic construct
GGVGKDTIS

SEQ ID NO: 8712 - protein, 9 aa, synthetic construct
GGEGSDIYV

SEQ ID NO: 8713 - protein, 9 aa, synthetic construct
GGEGSDKLY

SEQ ID NO: 8714 - protein, 9 aa, synthetic construct
GGVGKDKLY

SEQ ID NO: 8715 - protein, 9 aa, synthetic construct
GGEGNDTVL

SEQ ID NO: 8716 - protein, 9 aa, synthetic construct
GGEGADVFI

SEQ ID NO: 8717 - protein, 9 aa, synthetic construct
GGNGDDLLY

SEQ ID NO: 8718 - protein, 9 aa, synthetic construct
GGEGNDEIH

SEQ ID NO: 8719 - protein, 9 aa, synthetic construct
GGDGDDVVE

SEQ ID NO: 8720 - protein, 9 aa, synthetic construct
GGMGNDTLI

SEQ ID NO: 8721 - protein, 9 aa, synthetic construct
GGAGDDIIK

SEQ ID NO: 8722 - protein, 9 aa, synthetic construct
GGTGADEFI

SEQ ID NO: 8723 - protein, 9 aa, synthetic construct
GGIGADVLQ

SEQ ID NO: 8724 - protein, 9 aa, synthetic construct
GGVGTDTAS

SEQ ID NO: 8725 - protein, 9 aa, synthetic construct
GGTGADVVF

SEQ ID NO: 8726 - protein, 9 aa, synthetic construct
GGNGDDFLG

SEQ ID NO: 8727 - protein, 9 aa, synthetic construct
GGAGGDSLF

SEQ ID NO: 8728 - protein, 9 aa, synthetic construct
GGAGGDSLI

SEQ ID NO: 8729 - protein, 9 aa, synthetic construct
GGAGGDSLV

SEQ ID NO: 8730 - protein, 9 aa, synthetic construct
GGDGRDSAD

SEQ ID NO: 8731 - protein, 9 aa, synthetic construct
GGNGADVLI

SEQ ID NO: 8732 - protein, 9 aa, synthetic construct
GGNGADVLN

SEQ ID NO: 8733 - protein, 9 aa, synthetic construct
GGTGADVLF

SEQ ID NO: 8734 - protein, 9 aa, synthetic construct
GGDGRDRLE

SEQ ID NO: 8735 - protein, 9 aa, synthetic construct
GGTGADVMA

SEQ ID NO: 8736 - protein, 9 aa, synthetic construct
GGTGADVME

SEQ ID NO: 8737 - protein, 9 aa, synthetic construct
GGAGHDVLI

SEQ ID NO: 8738 - protein, 9 aa, synthetic construct
GGLGSDTLA

SEQ ID NO: 8739 - protein, 9 aa, synthetic construct
GGAGGDWLE

SEQ ID NO: 8740 - protein, 9 aa, synthetic construct
GGDGDDQIS

SEQ ID NO: 8741 - protein, 9 aa, synthetic construct
GGAGGDTLV

SEQ ID NO: 8742 - protein, 9 aa, synthetic construct
GGTGGDLMT

SEQ ID NO: 8743 - protein, 9 aa, synthetic construct
GGIGNDQLY

SEQ ID NO: 8744 - protein, 9 aa, synthetic construct
GGAGGDVFR

SEQ ID NO: 8745 - protein, 9 aa, synthetic construct
GGAGGDVLA

SEQ ID NO: 8746 - protein, 9 aa, synthetic construct
GGGGNDTVA

SEQ ID NO: 8747 - protein, 9 aa, synthetic construct
GGTGFDTLS

SEQ ID NO: 8748 - protein, 9 aa, synthetic construct
GGFGADQLR

SEQ ID NO: 8749 - protein, 9 aa, synthetic construct
GGAGGDVLR

SEQ ID NO: 8750 - protein, 9 aa, synthetic construct
GGEGADTLQ

SEQ ID NO: 8751 - protein, 9 aa, synthetic construct
GGEGADTLR

SEQ ID NO: 8752 - protein, 9 aa, synthetic construct
GGTGADVFI

SEQ ID NO: 8753 - protein, 9 aa, synthetic construct
GGNGADVIN

SEQ ID NO: 8754 - protein, 9 aa, synthetic construct
GGNGDDFLN

SEQ ID NO: 8755 - protein, 9 aa, synthetic construct
GGEGNDLIL

SEQ ID NO: 8756 - protein, 9 aa, synthetic construct
GGDGRDTLT

SEQ ID NO: 8757 - protein, 9 aa, synthetic construct
GGTGKDAFV

SEQ ID NO: 8758 - protein, 9 aa, synthetic construct
GGDGRDTLF

SEQ ID NO: 8759 - protein, 9 aa, synthetic construct
GGTGIDTAD

SEQ ID NO: 8760 - protein, 9 aa, synthetic construct
GGTGADTAS

SEQ ID NO: 8761 - protein, 9 aa, synthetic construct
GGGGNDYID

SEQ ID NO: 8762 - protein, 9 aa, synthetic construct
GGAGGDKLD

SEQ ID NO: 8763 - protein, 9 aa, synthetic construct
GGLGSDVLT

SEQ ID NO: 8764 - protein, 9 aa, synthetic construct
GGEGNDLMT

SEQ ID NO: 8765 - protein, 9 aa, synthetic construct
GGDGRDTFV

SEQ ID NO: 8766 - protein, 9 aa, synthetic construct
GGTGADTIF

SEQ ID NO: 8767 - protein, 9 aa, synthetic construct
GGTGADTIL

SEQ ID NO: 8768 - protein, 9 aa, synthetic construct
GGAGGDLLN

SEQ ID NO: 8769 - protein, 9 aa, synthetic construct
GGAGGDLLV

SEQ ID NO: 8770 - protein, 9 aa, synthetic construct
GGAGGDLVN

SEQ ID NO: 8771 - protein, 9 aa, synthetic construct
GGTGHDVLS

SEQ ID NO: 8772 - protein, 9 aa, synthetic construct
GGIGNDILS

SEQ ID NO: 8773 - protein, 9 aa, synthetic construct
GGTGHDTLV

SEQ ID NO: 8774 - protein, 9 aa, synthetic construct
GGIGNDIYI

SEQ ID NO: 8775 - protein, 9 aa, synthetic construct
GGTGADTMD

SEQ ID NO: 8776 - protein, 9 aa, synthetic construct
GGGGNDWLT

SEQ ID NO: 8777 - protein, 9 aa, synthetic construct
GGTGHDRLF

SEQ ID NO: 8778 - protein, 9 aa, synthetic construct
GGTGADTVD

SEQ ID NO: 8779 - protein, 9 aa, synthetic construct
GGTGHDRLD

SEQ ID NO: 8780 - protein, 9 aa, synthetic construct
GGAGGDRLE

SEQ ID NO: 8781 - protein, 9 aa, synthetic construct
GGFGADRLA

SEQ ID NO: 8782 - protein, 9 aa, synthetic construct
GGIGNDSLE

SEQ ID NO: 8783 - protein, 9 aa, synthetic construct
GGEGNDMLH

SEQ ID NO: 8784 - protein, 9 aa, synthetic construct
GGTGDDLVY

SEQ ID NO: 8785 - protein, 9 aa, synthetic construct
GGFGDDILD

SEQ ID NO: 8786 - protein, 9 aa, synthetic construct
GGTGDDELS

SEQ ID NO: 8787 - protein, 9 aa, synthetic construct
GGGGNDVIR

SEQ ID NO: 8788 - protein, 9 aa, synthetic construct
GGTGDDRLN

SEQ ID NO: 8789 - protein, 9 aa, synthetic construct
GGDGRDDLF

SEQ ID NO: 8790 - protein, 9 aa, synthetic construct
GGAGHDLLN

SEQ ID NO: 8791 - protein, 9 aa, synthetic construct
GGTGDDRIS

SEQ ID NO: 8792 - protein, 9 aa, synthetic construct
GGTGDDFIG

SEQ ID NO: 8793 - protein, 9 aa, synthetic construct
GGDGDDQLQ

SEQ ID NO: 8794 - protein, 9 aa, synthetic construct
GGTGDDNLL

SEQ ID NO: 8795 - protein, 9 aa, synthetic construct
GGTGDDNLF

SEQ ID NO: 8796 - protein, 9 aa, synthetic construct
GGNGDDDIS

SEQ ID NO: 8797 - protein, 9 aa, synthetic construct
GGTGDDLMI

SEQ ID NO: 8798 - protein, 9 aa, synthetic construct
GGAGGDYFI

SEQ ID NO: 8799 - protein, 9 aa, synthetic construct
GGTGDDLLT

SEQ ID NO: 8800 - protein, 9 aa, synthetic construct
GGTGDDLLQ

SEQ ID NO: 8801 - protein, 9 aa, synthetic construct
GGTGDDLLK

SEQ ID NO: 8802 - protein, 9 aa, synthetic construct
GGDGRDELQ

SEQ ID NO: 8803 - protein, 9 aa, synthetic construct
GGEGNDIIT

SEQ ID NO: 8804 - protein, 9 aa, synthetic construct
GGEGNDIIS

SEQ ID NO: 8805 - protein, 9 aa, synthetic construct
GGAGHDRLN

SEQ ID NO: 8806 - protein, 9 aa, synthetic construct
GGIGQDTVI

SEQ ID NO: 8807 - protein, 9 aa, synthetic construct
GGAGHDSLT

SEQ ID NO: 8808 - protein, 9 aa, synthetic construct
GGTGDDIMR

SEQ ID NO: 8809 - protein, 9 aa, synthetic construct
GGTGDDILK

SEQ ID NO: 8810 - protein, 9 aa, synthetic construct
GGTGDDIIV

SEQ ID NO: 8811 - protein, 9 aa, synthetic construct
GGIGNDVMI

SEQ ID NO: 8812 - protein, 9 aa, synthetic construct
GGTGDDRYI

SEQ ID NO: 8813 - protein, 9 aa, synthetic construct
GGLGSDTYF

SEQ ID NO: 8814 - protein, 9 aa, synthetic construct
GGAGHDTIY

SEQ ID NO: 8815 - protein, 9 aa, synthetic construct
GGTGEDVLY

SEQ ID NO: 8816 - protein, 9 aa, synthetic construct
GGIGNDSLV

SEQ ID NO: 8817 - protein, 9 aa, synthetic construct
GGDGDDRIL

SEQ ID NO: 8818 - protein, 9 aa, synthetic construct
GGGGNDTVN

SEQ ID NO: 8819 - protein, 9 aa, synthetic construct
GGAGGDYLD

SEQ ID NO: 8820 - protein, 9 aa, synthetic construct
GGLGSDVIE

SEQ ID NO: 8821 - protein, 9 aa, synthetic construct
GGTGEDTIH

SEQ ID NO: 8822 - protein, 9 aa, synthetic construct
GGFGADTFV

SEQ ID NO: 8823 - protein, 9 aa, synthetic construct
GGTGEDKFI

SEQ ID NO: 8824 - protein, 9 aa, synthetic construct
GGEGNDKID

SEQ ID NO: 8825 - protein, 9 aa, synthetic construct
GGDGRDALD

SEQ ID NO: 8826 - protein, 9 aa, synthetic construct
GGFGADTLR

SEQ ID NO: 8827 - protein, 9 aa, synthetic construct
GGIGNDTLG

SEQ ID NO: 8828 - protein, 9 aa, synthetic construct
GGTGDDALH

SEQ ID NO: 8829 - protein, 9 aa, synthetic construct
GGEGNDIYI

SEQ ID NO: 8830 - protein, 9 aa, synthetic construct
GGIGNDTLM

SEQ ID NO: 8831 - protein, 9 aa, synthetic construct
GGGGNDTVT

SEQ ID NO: 8832 - protein, 9 aa, synthetic construct
GGTGDDWLF

SEQ ID NO: 8833 - protein, 9 aa, synthetic construct
GGAGHDILH

SEQ ID NO: 8834 - protein, 9 aa, synthetic construct
GGTGDDVIR

SEQ ID NO: 8835 - protein, 9 aa, synthetic construct
GGAGHDTLH

SEQ ID NO: 8836 - protein, 9 aa, synthetic construct
GGTGDDTMS

SEQ ID NO: 8837 - protein, 9 aa, synthetic construct
GGEGNDIVE

SEQ ID NO: 8838 - protein, 9 aa, synthetic construct
GGTGDDTIE

SEQ ID NO: 8839 - protein, 9 aa, synthetic construct
GGGGNDVIT

SEQ ID NO: 8840 - protein, 9 aa, synthetic construct
GGAGHDWLS

SEQ ID NO: 8841 - protein, 9 aa, synthetic construct
GGEGNDMLI

SEQ ID NO: 8842 - protein, 9 aa, synthetic construct
GGTGRDVLS

SEQ ID NO: 8843 - protein, 9 aa, synthetic construct
GGTGNDTVN

SEQ ID NO: 8844 - protein, 9 aa, synthetic construct
GGDGQDRLF

SEQ ID NO: 8845 - protein, 9 aa, synthetic construct
GGTGNDYLY

SEQ ID NO: 8846 - protein, 9 aa, synthetic construct
GGTGNDYIS

SEQ ID NO: 8847 - protein, 9 aa, synthetic construct
GGTGNDWLY

SEQ ID NO: 8848 - protein, 9 aa, synthetic construct
GGIGDDTID

SEQ ID NO: 8849 - protein, 9 aa, synthetic construct
GGTGNDWIF

SEQ ID NO: 8850 - protein, 9 aa, synthetic construct
GGNGADLLN

SEQ ID NO: 8851 - protein, 9 aa, synthetic construct
GGTGNDVYI

SEQ ID NO: 8852 - protein, 9 aa, synthetic construct
GGTGNDVMT

SEQ ID NO: 8853 - protein, 9 aa, synthetic construct
GGTGNDVIS

SEQ ID NO: 8854 - protein, 9 aa, synthetic construct
GGTGNDVFY

SEQ ID NO: 8855 - protein, 9 aa, synthetic construct
GGEGTDTIT

SEQ ID NO: 8856 - protein, 9 aa, synthetic construct
GGTGNDTFL

SEQ ID NO: 8857 - protein, 9 aa, synthetic construct
GGFGDDRLI

SEQ ID NO: 8858 - protein, 9 aa, synthetic construct
GGAGEDVLL

SEQ ID NO: 8859 - protein, 9 aa, synthetic construct
GGTGNDSMT

SEQ ID NO: 8860 - protein, 9 aa, synthetic construct
GGAGEDVLN

SEQ ID NO: 8861 - protein, 9 aa, synthetic construct
GGTGNDSMD

SEQ ID NO: 8862 - protein, 9 aa, synthetic construct
GGTGNDSLW

SEQ ID NO: 8863 - protein, 9 aa, synthetic construct
GGTGNDSIV

SEQ ID NO: 8864 - protein, 9 aa, synthetic construct
GGAGEDVVR

SEQ ID NO: 8865 - protein, 9 aa, synthetic construct
GGAGEDVVV

SEQ ID NO: 8866 - protein, 9 aa, synthetic construct
GGTGNDRIT

SEQ ID NO: 8867 - protein, 9 aa, synthetic construct
GGTGNDRIH

SEQ ID NO: 8868 - protein, 9 aa, synthetic construct
GGTGNDQMG

SEQ ID NO: 8869 - protein, 9 aa, synthetic construct
GGTGNDQLQ

SEQ ID NO: 8870 - protein, 9 aa, synthetic construct
GGNGADKLY

SEQ ID NO: 8871 - protein, 9 aa, synthetic construct
GGIGDDNLI

SEQ ID NO: 8872 - protein, 9 aa, synthetic construct
GGDGDDTFL

SEQ ID NO: 8873 - protein, 9 aa, synthetic construct
GGIGDDMLI

SEQ ID NO: 8874 - protein, 9 aa, synthetic construct
GGIGTDTLY

SEQ ID NO: 8875 - protein, 9 aa, synthetic construct
GGAGDDYLL

SEQ ID NO: 8876 - protein, 9 aa, synthetic construct
GGAGDDYLR

SEQ ID NO: 8877 - protein, 9 aa, synthetic construct
GGDGDDTIW

SEQ ID NO: 8878 - protein, 9 aa, synthetic construct
GGEGADRLY

SEQ ID NO: 8879 - protein, 9 aa, synthetic construct
GGTGRDRLL

SEQ ID NO: 8880 - protein, 9 aa, synthetic construct
GGDGFDTLD

SEQ ID NO: 8881 - protein, 9 aa, synthetic construct
GGDGDDTIK

SEQ ID NO: 8882 - protein, 9 aa, synthetic construct
GGGGQDVFV

SEQ ID NO: 8883 - protein, 9 aa, synthetic construct
GGAGEDELL

SEQ ID NO: 8884 - protein, 9 aa, synthetic construct
GGDGDDTIH

SEQ ID NO: 8885 - protein, 9 aa, synthetic construct
GGNGADIFR

SEQ ID NO: 8886 - protein, 9 aa, synthetic construct
GGDGSDRLL

SEQ ID NO: 8887 - protein, 9 aa, synthetic construct
GGEGNDSLV

SEQ ID NO: 8888 - protein, 9 aa, synthetic construct
GGAGEDIIY

SEQ ID NO: 8889 - protein, 9 aa, synthetic construct
GGNGADILL

SEQ ID NO: 8890 - protein, 9 aa, synthetic construct
GGEGNDSLE

SEQ ID NO: 8891 - protein, 9 aa, synthetic construct
GGNGADILN

SEQ ID NO: 8892 - protein, 9 aa, synthetic construct
GGGGQDTLT

SEQ ID NO: 8893 - protein, 9 aa, synthetic construct
GGTGRDAYY

SEQ ID NO: 8894 - protein, 9 aa, synthetic construct
GGEGNDSIY

SEQ ID NO: 8895 - protein, 9 aa, synthetic construct
GGGGQDTLS

SEQ ID NO: 8896 - protein, 9 aa, synthetic construct
GGAGEDLLI

SEQ ID NO: 8897 - protein, 9 aa, synthetic construct
GGEGDDQLT

SEQ ID NO: 8898 - protein, 9 aa, synthetic construct
GGAGEDLVT

SEQ ID NO: 8899 - protein, 9 aa, synthetic construct
GGFGDDRLY

SEQ ID NO: 8900 - protein, 9 aa, synthetic construct
GGIGDDVMQ

SEQ ID NO: 8901 - protein, 9 aa, synthetic construct
GGAGGDFLD

SEQ ID NO: 8902 - protein, 9 aa, synthetic construct
GGDGRDYLE

SEQ ID NO: 8903 - protein, 9 aa, synthetic construct
GGIGHDSLT

SEQ ID NO: 8904 - protein, 9 aa, synthetic construct
GGIGHDSLV

SEQ ID NO: 8905 - protein, 9 aa, synthetic construct
GGEGADTFI

SEQ ID NO: 8906 - protein, 9 aa, synthetic construct
GGTGNDALI

SEQ ID NO: 8907 - protein, 9 aa, synthetic construct
GGEGVDTLT

SEQ ID NO: 8908 - protein, 9 aa, synthetic construct
GGIGHDTLS

SEQ ID NO: 8909 - protein, 9 aa, synthetic construct
GGIGHDVLN

SEQ ID NO: 8910 - protein, 9 aa, synthetic construct
GGDGSDALN

SEQ ID NO: 8911 - protein, 9 aa, synthetic construct
GGNGADSLF

SEQ ID NO: 8912 - protein, 9 aa, synthetic construct
GGDGDDSIF

SEQ ID NO: 8913 - protein, 9 aa, synthetic construct
GGTGADRIY

SEQ ID NO: 8914 - protein, 9 aa, synthetic construct
GGIGIDTLV

SEQ ID NO: 8915 - protein, 9 aa, synthetic construct
GGEGNDNLT

SEQ ID NO: 8916 - protein, 9 aa, synthetic construct
GGTGNDNLT

SEQ ID NO: 8917 - protein, 9 aa, synthetic construct
GGEGNDNLQ

SEQ ID NO: 8918 - protein, 9 aa, synthetic construct
GGDGRDWLL

SEQ ID NO: 8919 - protein, 9 aa, synthetic construct
GGTGADRML

SEQ ID NO: 8920 - protein, 9 aa, synthetic construct
GGNGADTID

SEQ ID NO: 8921 - protein, 9 aa, synthetic construct
GGTGKDTLV

SEQ ID NO: 8922 - protein, 9 aa, synthetic construct
GGTGKDTLK

SEQ ID NO: 8923 - protein, 9 aa, synthetic construct
GGTGADRMV

SEQ ID NO: 8924 - protein, 9 aa, synthetic construct
GGGGNDYLI

SEQ ID NO: 8925 - protein, 9 aa, synthetic construct
GGTGKDQMT

SEQ ID NO: 8926 - protein, 9 aa, synthetic construct
GGDGDDQID

SEQ ID NO: 8927 - protein, 9 aa, synthetic construct
GGTGKDKLY

SEQ ID NO: 8928 - protein, 9 aa, synthetic construct
GGTGADSLL

SEQ ID NO: 8929 - protein, 9 aa, synthetic construct
GGDGDDSIV

SEQ ID NO: 8930 - protein, 9 aa, synthetic construct
GGTGNDDLS

SEQ ID NO: 8931 - protein, 9 aa, synthetic construct
GGDGDDSLA

SEQ ID NO: 8932 - protein, 9 aa, synthetic construct
GGTGADQLT

SEQ ID NO: 8933 - protein, 9 aa, synthetic construct
GGDGDDSVD

SEQ ID NO: 8934 - protein, 9 aa, synthetic construct
GGFGDDRLF

SEQ ID NO: 8935 - protein, 9 aa, synthetic construct
GGTGNDNIG

SEQ ID NO: 8936 - protein, 9 aa, synthetic construct
GGTGNDMLT

SEQ ID NO: 8937 - protein, 9 aa, synthetic construct
GGTGNDMLL

SEQ ID NO: 8938 - protein, 9 aa, synthetic construct
GGTGNDLMR

SEQ ID NO: 8939 - protein, 9 aa, synthetic construct
GGTGNDLMQ

SEQ ID NO: 8940 - protein, 9 aa, synthetic construct
GGIGEDSFI

SEQ ID NO: 8941 - protein, 9 aa, synthetic construct
GGDGSDIYF

SEQ ID NO: 8942 - protein, 9 aa, synthetic construct
GGTGNDLIE

SEQ ID NO: 8943 - protein, 9 aa, synthetic construct
GGTGNDLAV

SEQ ID NO: 8944 - protein, 9 aa, synthetic construct
GGTGNDKVY

SEQ ID NO: 8945 - protein, 9 aa, synthetic construct
GGIGEDWLE

SEQ ID NO: 8946 - protein, 9 aa, synthetic construct
GGNGDDHLS

SEQ ID NO: 8947 - protein, 9 aa, synthetic construct
GGTGNDKIY

SEQ ID NO: 8948 - protein, 9 aa, synthetic construct
GGTGNDKIF

SEQ ID NO: 8949 - protein, 9 aa, synthetic construct
GGDGDDSLW

SEQ ID NO: 8950 - protein, 9 aa, synthetic construct
GGTGNDIIS

SEQ ID NO: 8951 - protein, 9 aa, synthetic construct
GGDGDDSLQ

SEQ ID NO: 8952 - protein, 9 aa, synthetic construct
GGNGADRLF

SEQ ID NO: 8953 - protein, 9 aa, synthetic construct
GGIGSDTLD

SEQ ID NO: 8954 - protein, 9 aa, synthetic construct
GGAGFDQLT

SEQ ID NO: 8955 - protein, 9 aa, synthetic construct
GGEGNDQLS

SEQ ID NO: 8956 - protein, 9 aa, synthetic construct
GGTGNDELS

SEQ ID NO: 8957 - protein, 9 aa, synthetic construct
GGEGADTAS

SEQ ID NO: 8958 - protein, 9 aa, synthetic construct
GGVGTDRAS

SEQ ID NO: 8959 - protein, 9 aa, synthetic construct
GGAGHDSIT

SEQ ID NO: 8960 - protein, 9 aa, synthetic construct
GGYGLDFLN

SEQ ID NO: 8961 - protein, 9 aa, synthetic construct
GGGGRDYIV

SEQ ID NO: 8962 - protein, 9 aa, synthetic construct
GGGGSDLLR

SEQ ID NO: 8963 - protein, 9 aa, synthetic construct
GGAGADKFK

SEQ ID NO: 8964 - protein, 9 aa, synthetic construct
GGGGVDLLN

SEQ ID NO: 8965 - protein, 9 aa, synthetic construct
GGAGADMFV

SEQ ID NO: 8966 - protein, 9 aa, synthetic construct
GGGGSDTYI

SEQ ID NO: 8967 - protein, 9 aa, synthetic construct
GGEGQDTLL

SEQ ID NO: 8968 - protein, 9 aa, synthetic construct
GGSGSDLLE

SEQ ID NO: 8969 - protein, 9 aa, synthetic construct
GGGGSDLLD

SEQ ID NO: 8970 - protein, 9 aa, synthetic construct
GGDGEDVLV

SEQ ID NO: 8971 - protein, 9 aa, synthetic construct
GGAGADDLF

SEQ ID NO: 8972 - protein, 9 aa, synthetic construct
GGAGADDLH

SEQ ID NO: 8973 - protein, 9 aa, synthetic construct
GGAGADSMF

SEQ ID NO: 8974 - protein, 9 aa, synthetic construct
GGAGADIIT

SEQ ID NO: 8975 - protein, 9 aa, synthetic construct
GGGGSDSIT

SEQ ID NO: 8976 - protein, 9 aa, synthetic construct
GGFGHDRMN

SEQ ID NO: 8977 - protein, 9 aa, synthetic construct
GGSGSDLLF

SEQ ID NO: 8978 - protein, 9 aa, synthetic construct
GGDGNDYLL

SEQ ID NO: 8979 - protein, 9 aa, synthetic construct
GGSGRDVLS

SEQ ID NO: 8980 - protein, 9 aa, synthetic construct
GGDGNDYLK

SEQ ID NO: 8981 - protein, 9 aa, synthetic construct
GGGGHDFLI

SEQ ID NO: 8982 - protein, 9 aa, synthetic construct
GGEGNDYID

SEQ ID NO: 8983 - protein, 9 aa, synthetic construct
GGWGDDVVI

SEQ ID NO: 8984 - protein, 9 aa, synthetic construct
GGEGDDSLE

SEQ ID NO: 8985 - protein, 9 aa, synthetic construct
GGSGRDTLK

SEQ ID NO: 8986 - protein, 9 aa, synthetic construct
GGGGSDRLT

SEQ ID NO: 8987 - protein, 9 aa, synthetic construct
GGWGEDTLD

SEQ ID NO: 8988 - protein, 9 aa, synthetic construct
GGWGEDRIA

SEQ ID NO: 8989 - protein, 9 aa, synthetic construct
GGGGNDRLQ

SEQ ID NO: 8990 - protein, 9 aa, synthetic construct
GGYGDDTLT

SEQ ID NO: 8991 - protein, 9 aa, synthetic construct
GGMGDDVLV

SEQ ID NO: 8992 - protein, 9 aa, synthetic construct
GGAGADIII

SEQ ID NO: 8993 - protein, 9 aa, synthetic construct
GGSGRDTIT

SEQ ID NO: 8994 - protein, 9 aa, synthetic construct
GGAGADLMN

SEQ ID NO: 8995 - protein, 9 aa, synthetic construct
GGYGDDTLY

SEQ ID NO: 8996 - protein, 9 aa, synthetic construct
GGAGADVAA

SEQ ID NO: 8997 - protein, 9 aa, synthetic construct
GGGGSDELT

SEQ ID NO: 8998 - protein, 9 aa, synthetic construct
GGYGNDILR

SEQ ID NO: 8999 - protein, 9 aa, synthetic construct
GGSGSDILI

SEQ ID NO: 9000 - protein, 9 aa, synthetic construct
GGWGNDTLL

SEQ ID NO: 9001 - protein, 9 aa, synthetic construct
GGKGDDIIY

SEQ ID NO: 9002 - protein, 9 aa, synthetic construct
GGMGDDLLI

SEQ ID NO: 9003 - protein, 9 aa, synthetic construct
GGGGTDTLL

SEQ ID NO: 9004 - protein, 9 aa, synthetic construct
GGAGKDTMR

SEQ ID NO: 9005 - protein, 9 aa, synthetic construct
GGSGRDSLS

SEQ ID NO: 9006 - protein, 9 aa, synthetic construct
GGMGDDRLF

SEQ ID NO: 9007 - protein, 9 aa, synthetic construct
GGAGADNLN

SEQ ID NO: 9008 - protein, 9 aa, synthetic construct
GGAGADNLV

SEQ ID NO: 9009 - protein, 9 aa, synthetic construct
GGAGADTFE

SEQ ID NO: 9010 - protein, 9 aa, synthetic construct
GGDGVDTIY

SEQ ID NO: 9011 - protein, 9 aa, synthetic construct
GGAGADTFM

SEQ ID NO: 9012 - protein, 9 aa, synthetic construct
GGAGADTFN

SEQ ID NO: 9013 - protein, 9 aa, synthetic construct
GGAGADIMA

SEQ ID NO: 9014 - protein, 9 aa, synthetic construct
GGYGNDSLL

SEQ ID NO: 9015 - protein, 9 aa, synthetic construct
GGGGNDRLR

SEQ ID NO: 9016 - protein, 9 aa, synthetic construct
GGWGDDMLD

SEQ ID NO: 9017 - protein, 9 aa, synthetic construct
GGAGADIMD

SEQ ID NO: 9018 - protein, 9 aa, synthetic construct
GGEGRDTID

SEQ ID NO: 9019 - protein, 9 aa, synthetic construct
GGYGNDTLE

SEQ ID NO: 9020 - protein, 9 aa, synthetic construct
GGYGNDTIY

SEQ ID NO: 9021 - protein, 9 aa, synthetic construct
GGGGVDILD

SEQ ID NO: 9022 - protein, 9 aa, synthetic construct
GGAGADTIR

SEQ ID NO: 9023 - protein, 9 aa, synthetic construct
GGEGQDILT

SEQ ID NO: 9024 - protein, 9 aa, synthetic construct
GGEGNDALD

SEQ ID NO: 9025 - protein, 9 aa, synthetic construct
GGDGVDTIS

SEQ ID NO: 9026 - protein, 9 aa, synthetic construct
GGYGNDTID

SEQ ID NO: 9027 - protein, 9 aa, synthetic construct
GGNGDDRLD

SEQ ID NO: 9028 - protein, 9 aa, synthetic construct
GGAGADFLY

SEQ ID NO: 9029 - protein, 9 aa, synthetic construct
GGAGADIIY

SEQ ID NO: 9030 - protein, 9 aa, synthetic construct
GGAGADILM

SEQ ID NO: 9031 - protein, 9 aa, synthetic construct
GGAGADKAE

SEQ ID NO: 9032 - protein, 9 aa, synthetic construct
GGDGEDTLF

SEQ ID NO: 9033 - protein, 9 aa, synthetic construct
GGGGYDIID

SEQ ID NO: 9034 - protein, 9 aa, synthetic construct
GGEGDDRLR

SEQ ID NO: 9035 - protein, 9 aa, synthetic construct
GGDGVDTIA

SEQ ID NO: 9036 - protein, 9 aa, synthetic construct
GGAGKDRLI

SEQ ID NO: 9037 - protein, 9 aa, synthetic construct
GGEGDDRLG

SEQ ID NO: 9038 - protein, 9 aa, synthetic construct
GGEGQDVIQ

SEQ ID NO: 9039 - protein, 9 aa, synthetic construct
GGGGSDSVY

SEQ ID NO: 9040 - protein, 9 aa, synthetic construct
GGYGQDVLI

SEQ ID NO: 9041 - protein, 9 aa, synthetic construct
GGDGVDTLN

SEQ ID NO: 9042 - protein, 9 aa, synthetic construct
GGAGADELF

SEQ ID NO: 9043 - protein, 9 aa, synthetic construct
GGAGADMLV

SEQ ID NO: 9044 - protein, 9 aa, synthetic construct
GGAGADMMY

SEQ ID NO: 9045 - protein, 9 aa, synthetic construct
GGAGADILL

SEQ ID NO: 9046 - protein, 9 aa, synthetic construct
GGEGDDRFV

SEQ ID NO: 9047 - protein, 9 aa, synthetic construct
GGAGADNLI

SEQ ID NO: 9048 - protein, 9 aa, synthetic construct
GGAGADELT

SEQ ID NO: 9049 - protein, 9 aa, synthetic construct
GGAGADNLL

SEQ ID NO: 9050 - protein, 9 aa, synthetic construct
GGGGSDFLD

SEQ ID NO: 9051 - protein, 9 aa, synthetic construct
GGGGWDRLV

SEQ ID NO: 9052 - protein, 9 aa, synthetic construct
GGAGADRIN

SEQ ID NO: 9053 - protein, 9 aa, synthetic construct
GGAGKDQLY

SEQ ID NO: 9054 - protein, 9 aa, synthetic construct
GGYGYDILI

SEQ ID NO: 9055 - protein, 9 aa, synthetic construct
GGAGKDSYV

SEQ ID NO: 9056 - protein, 9 aa, synthetic construct
GGYGNDIIQ

SEQ ID NO: 9057 - protein, 9 aa, synthetic construct
GGWGKDTFY

SEQ ID NO: 9058 - protein, 9 aa, synthetic construct
GGAGADHFI

SEQ ID NO: 9059 - protein, 9 aa, synthetic construct
GGEGDDRIL

SEQ ID NO: 9060 - protein, 9 aa, synthetic construct
GGGGHDKLY

SEQ ID NO: 9061 - protein, 9 aa, synthetic construct
GGGGSDRID

SEQ ID NO: 9062 - protein, 9 aa, synthetic construct
GGEGADIID

SEQ ID NO: 9063 - protein, 9 aa, synthetic construct
GGAGADAMF

SEQ ID NO: 9064 - protein, 9 aa, synthetic construct
GGAGKDRID

SEQ ID NO: 9065 - protein, 9 aa, synthetic construct
GGGGVDSLF

SEQ ID NO: 9066 - protein, 9 aa, synthetic construct
GGAGADVIE

SEQ ID NO: 9067 - protein, 9 aa, synthetic construct
GGYGDDRLE

SEQ ID NO: 9068 - protein, 9 aa, synthetic construct
GGAGADSIA

SEQ ID NO: 9069 - protein, 9 aa, synthetic construct
GGGGSDVLL

SEQ ID NO: 9070 - protein, 9 aa, synthetic construct
GGDGYDRIS

SEQ ID NO: 9071 - protein, 9 aa, synthetic construct
GGEGDDRLH

SEQ ID NO: 9072 - protein, 9 aa, synthetic construct
GGYGVDTID

SEQ ID NO: 9073 - protein, 9 aa, synthetic construct
GGAGADHLF

SEQ ID NO: 9074 - protein, 9 aa, synthetic construct
GGGGYDTLY

SEQ ID NO: 9075 - protein, 9 aa, synthetic construct
GGYGDDTFH

SEQ ID NO: 9076 - protein, 9 aa, synthetic construct
GGMGDDQII

SEQ ID NO: 9077 - protein, 9 aa, synthetic construct
GGGGSDVLN

SEQ ID NO: 9078 - protein, 9 aa, synthetic construct
GGAGADKME

SEQ ID NO: 9079 - protein, 9 aa, synthetic construct
GGSGSDALR

SEQ ID NO: 9080 - protein, 9 aa, synthetic construct
GGGGRDVLA

SEQ ID NO: 9081 - protein, 9 aa, synthetic construct
GGYGVDKMT

SEQ ID NO: 9082 - protein, 9 aa, synthetic construct
GGEGQDQLL

SEQ ID NO: 9083 - protein, 9 aa, synthetic construct
GGDGEDTLY

SEQ ID NO: 9084 - protein, 9 aa, synthetic construct
GGAGKDTLK

SEQ ID NO: 9085 - protein, 9 aa, synthetic construct
GGDGVDSLY

SEQ ID NO: 9086 - protein, 9 aa, synthetic construct
GGAGADGLY

SEQ ID NO: 9087 - protein, 9 aa, synthetic construct
GGFGHDLVN

SEQ ID NO: 9088 - protein, 9 aa, synthetic construct
GGMGDDAMY

SEQ ID NO: 9089 - protein, 9 aa, synthetic construct
GGWGKDWLL

SEQ ID NO: 9090 - protein, 9 aa, synthetic construct
GGAGADHLY

SEQ ID NO: 9091 - protein, 9 aa, synthetic construct
GGAGADSIF

SEQ ID NO: 9092 - protein, 9 aa, synthetic construct
GGDGDDLVR

SEQ ID NO: 9093 - protein, 9 aa, synthetic construct
GGAGADRIA

SEQ ID NO: 9094 - protein, 9 aa, synthetic construct
GGKGADYID

SEQ ID NO: 9095 - protein, 9 aa, synthetic construct
GGAGADAMS

SEQ ID NO: 9096 - protein, 9 aa, synthetic construct
GGAGADAFD

SEQ ID NO: 9097 - protein, 9 aa, synthetic construct
GGRGSDTYL

SEQ ID NO: 9098 - protein, 9 aa, synthetic construct
GGSGADLIY

SEQ ID NO: 9099 - protein, 9 aa, synthetic construct
GGAGFDTMT

SEQ ID NO: 9100 - protein, 9 aa, synthetic construct
GGDGNDIIE

SEQ ID NO: 9101 - protein, 9 aa, synthetic construct
GGEGDDKLV

SEQ ID NO: 9102 - protein, 9 aa, synthetic construct
GGNGSDELT

SEQ ID NO: 9103 - protein, 9 aa, synthetic construct
GGEGHDVLL

SEQ ID NO: 9104 - protein, 9 aa, synthetic construct
GGTGNDKLN

SEQ ID NO: 9105 - protein, 9 aa, synthetic construct
GGNGSDTFL

SEQ ID NO: 9106 - protein, 9 aa, synthetic construct
GGDGDDSIR

SEQ ID NO: 9107 - protein, 9 aa, synthetic construct
GGEGVDTVD

SEQ ID NO: 9108 - protein, 9 aa, synthetic construct
GGDGADLLH

SEQ ID NO: 9109 - protein, 9 aa, synthetic construct
GGRGSDTLD

SEQ ID NO: 9110 - protein, 9 aa, synthetic construct
GGTGNDNID

SEQ ID NO: 9111 - protein, 9 aa, synthetic construct
GGDGNDLFL

SEQ ID NO: 9112 - protein, 9 aa, synthetic construct
GGNGADQIR

SEQ ID NO: 9113 - protein, 9 aa, synthetic construct
GGLGNDSVS

SEQ ID NO: 9114 - protein, 9 aa, synthetic construct
GGAGADIFA

SEQ ID NO: 9115 - protein, 9 aa, synthetic construct
GGKGTDAYY

SEQ ID NO: 9116 - protein, 9 aa, synthetic construct
GGDGNDIIA

SEQ ID NO: 9117 - protein, 9 aa, synthetic construct
GGGGPDTFI

SEQ ID NO: 9118 - protein, 9 aa, synthetic construct
GGRGSDLYQ

SEQ ID NO: 9119 - protein, 9 aa, synthetic construct
GGKGTDLLN

SEQ ID NO: 9120 - protein, 9 aa, synthetic construct
GGEGDDQIF

SEQ ID NO: 9121 - protein, 9 aa, synthetic construct
GGAGFDTLR

SEQ ID NO: 9122 - protein, 9 aa, synthetic construct
GGFGYDRIN

SEQ ID NO: 9123 - protein, 9 aa, synthetic construct
GGSGADLAR

SEQ ID NO: 9124 - protein, 9 aa, synthetic construct
GGLGRDVMT

SEQ ID NO: 9125 - protein, 9 aa, synthetic construct
GGIGIDALN

SEQ ID NO: 9126 - protein, 9 aa, synthetic construct
GGEGNDRIL

SEQ ID NO: 9127 - protein, 9 aa, synthetic construct
GGMGDDIYV

SEQ ID NO: 9128 - protein, 9 aa, synthetic construct
GGEGADSLY

SEQ ID NO: 9129 - protein, 9 aa, synthetic construct
GGTGNDLME

SEQ ID NO: 9130 - protein, 9 aa, synthetic construct
GGTGNDLLQ

SEQ ID NO: 9131 - protein, 9 aa, synthetic construct
GGRGSDKLR

SEQ ID NO: 9132 - protein, 9 aa, synthetic construct
GGNGSDELY

SEQ ID NO: 9133 - protein, 9 aa, synthetic construct
GGDGADLIT

SEQ ID NO: 9134 - protein, 9 aa, synthetic construct
GGDGNDLFR

SEQ ID NO: 9135 - protein, 9 aa, synthetic construct
GGRGSDRLD

SEQ ID NO: 9136 - protein, 9 aa, synthetic construct
GGRGSDVLD

SEQ ID NO: 9137 - protein, 9 aa, synthetic construct
GGTGNDLLH

SEQ ID NO: 9138 - protein, 9 aa, synthetic construct
GGAGPDLLY

SEQ ID NO: 9139 - protein, 9 aa, synthetic construct
GGDGDDSIN

SEQ ID NO: 9140 - protein, 9 aa, synthetic construct
GGNGNDRMF

SEQ ID NO: 9141 - protein, 9 aa, synthetic construct
GGSGADKLS

SEQ ID NO: 9142 - protein, 9 aa, synthetic construct
GGDGDDSIQ

SEQ ID NO: 9143 - protein, 9 aa, synthetic construct
GGTGNDLFL

SEQ ID NO: 9144 - protein, 9 aa, synthetic construct
GGNGSDRMF

SEQ ID NO: 9145 - protein, 9 aa, synthetic construct
GGSGADLFA

SEQ ID NO: 9146 - protein, 9 aa, synthetic construct
GGGGNDLLK

SEQ ID NO: 9147 - protein, 9 aa, synthetic construct
GGTGNDELW

SEQ ID NO: 9148 - protein, 9 aa, synthetic construct
GGIGFDSLF

SEQ ID NO: 9149 - protein, 9 aa, synthetic construct
GGRGSDVLE

SEQ ID NO: 9150 - protein, 9 aa, synthetic construct
GGTGNDDLY

SEQ ID NO: 9151 - protein, 9 aa, synthetic construct
GGNGSDKLS

SEQ ID NO: 9152 - protein, 9 aa, synthetic construct
GGNGSDKLF

SEQ ID NO: 9153 - protein, 9 aa, synthetic construct
GGKGSDSYF

SEQ ID NO: 9154 - protein, 9 aa, synthetic construct
GGLGNDTAF

SEQ ID NO: 9155 - protein, 9 aa, synthetic construct
GGRGYDILI

SEQ ID NO: 9156 - protein, 9 aa, synthetic construct
GGEGADYLY

SEQ ID NO: 9157 - protein, 9 aa, synthetic construct
GGLGPDAFA

SEQ ID NO: 9158 - protein, 9 aa, synthetic construct
GGAGADIIL

SEQ ID NO: 9159 - protein, 9 aa, synthetic construct
GGAGADIMN

SEQ ID NO: 9160 - protein, 9 aa, synthetic construct
GGRGWDVLD

SEQ ID NO: 9161 - protein, 9 aa, synthetic construct
GGTGNDHLF

SEQ ID NO: 9162 - protein, 9 aa, synthetic construct
GGGGDDYLG

SEQ ID NO: 9163 - protein, 9 aa, synthetic construct
GGAGNDWLT

SEQ ID NO: 9164 - protein, 9 aa, synthetic construct
GGDGGDLLR

SEQ ID NO: 9165 - protein, 9 aa, synthetic construct
GGSGADFLN

SEQ ID NO: 9166 - protein, 9 aa, synthetic construct
GGEGDDMLF

SEQ ID NO: 9167 - protein, 9 aa, synthetic construct
GGKGSDVLT

SEQ ID NO: 9168 - protein, 9 aa, synthetic construct
GGAGNDWIF

SEQ ID NO: 9169 - protein, 9 aa, synthetic construct
GGTGNDELN

SEQ ID NO: 9170 - protein, 9 aa, synthetic construct
GGIGHDALY

SEQ ID NO: 9171 - protein, 9 aa, synthetic construct
GGSGADEIA

SEQ ID NO: 9172 - protein, 9 aa, synthetic construct
GGTGNDFIH

SEQ ID NO: 9173 - protein, 9 aa, synthetic construct
GGNGADRLV

SEQ ID NO: 9174 - protein, 9 aa, synthetic construct
GGAGADIIE

SEQ ID NO: 9175 - protein, 9 aa, synthetic construct
GGFGTDSMD

SEQ ID NO: 9176 - protein, 9 aa, synthetic construct
GGTGNDFVT

SEQ ID NO: 9177 - protein, 9 aa, synthetic construct
GGSGADDLF

SEQ ID NO: 9178 - protein, 9 aa, synthetic construct
GGAGNDWIS

SEQ ID NO: 9179 - protein, 9 aa, synthetic construct
GGNGSDKLY

SEQ ID NO: 9180 - protein, 9 aa, synthetic construct
GGSGADALQ

SEQ ID NO: 9181 - protein, 9 aa, synthetic construct
GGSGADALL

SEQ ID NO: 9182 - protein, 9 aa, synthetic construct
GGAGNDVVY

SEQ ID NO: 9183 - protein, 9 aa, synthetic construct
GGAGNDWMD

SEQ ID NO: 9184 - protein, 9 aa, synthetic construct
GGLGNDTFH

SEQ ID NO: 9185 - protein, 9 aa, synthetic construct
GGRGVDTLI

SEQ ID NO: 9186 - protein, 9 aa, synthetic construct
GGAGNDYMH

SEQ ID NO: 9187 - protein, 9 aa, synthetic construct
GGAGFDLAI

SEQ ID NO: 9188 - protein, 9 aa, synthetic construct
GGKGSDTYY

SEQ ID NO: 9189 - protein, 9 aa, synthetic construct
GGDGDDSMD

SEQ ID NO: 9190 - protein, 9 aa, synthetic construct
GGSGADILL

SEQ ID NO: 9191 - protein, 9 aa, synthetic construct
GGDGNDIVI

SEQ ID NO: 9192 - protein, 9 aa, synthetic construct
GGEGDDLFQ

SEQ ID NO: 9193 - protein, 9 aa, synthetic construct
GGTGNDIYW

SEQ ID NO: 9194 - protein, 9 aa, synthetic construct
GGKGSDTLD

SEQ ID NO: 9195 - protein, 9 aa, synthetic construct
GGEGADTFE

SEQ ID NO: 9196 - protein, 9 aa, synthetic construct
GGDGEDRLE

SEQ ID NO: 9197 - protein, 9 aa, synthetic construct
GGAGADIFD

SEQ ID NO: 9198 - protein, 9 aa, synthetic construct
GGAGNDYVN

SEQ ID NO: 9199 - protein, 9 aa, synthetic construct
GGEGNDQIT

SEQ ID NO: 9200 - protein, 9 aa, synthetic construct
GGLGNDTFT

SEQ ID NO: 9201 - protein, 9 aa, synthetic construct
GGAGFDLAV

SEQ ID NO: 9202 - protein, 9 aa, synthetic construct
GGDGADMLD

SEQ ID NO: 9203 - protein, 9 aa, synthetic construct
GGAGADIFT

SEQ ID NO: 9204 - protein, 9 aa, synthetic construct
GGTGNDAYV

SEQ ID NO: 9205 - protein, 9 aa, synthetic construct
GGNGADRFF

SEQ ID NO: 9206 - protein, 9 aa, synthetic construct
GGAGFDSLN

SEQ ID NO: 9207 - protein, 9 aa, synthetic construct
GGNGADRFV

SEQ ID NO: 9208 - protein, 9 aa, synthetic construct
GGAGNDYII

SEQ ID NO: 9209 - protein, 9 aa, synthetic construct
GGTGNDIIE

SEQ ID NO: 9210 - protein, 9 aa, synthetic construct
GGSGADIID

SEQ ID NO: 9211 - protein, 9 aa, synthetic construct
GGTGNDIFK

SEQ ID NO: 9212 - protein, 9 aa, synthetic construct
GGFGVDHLF

SEQ ID NO: 9213 - protein, 9 aa, synthetic construct
GGGGQDILW

SEQ ID NO: 9214 - protein, 9 aa, synthetic construct
GGTGNDDLD

SEQ ID NO: 9215 - protein, 9 aa, synthetic construct
GGAGNDVMR

SEQ ID NO: 9216 - protein, 9 aa, synthetic construct
GGAGNDVMY

SEQ ID NO: 9217 - protein, 9 aa, synthetic construct
GGAGFDLLY

SEQ ID NO: 9218 - protein, 9 aa, synthetic construct
GGNGGDFIV

SEQ ID NO: 9219 - protein, 9 aa, synthetic construct
GGNGNDKIW

SEQ ID NO: 9220 - protein, 9 aa, synthetic construct
GGDGADLIE

SEQ ID NO: 9221 - protein, 9 aa, synthetic construct
GGNGADKLI

SEQ ID NO: 9222 - protein, 9 aa, synthetic construct
GGRGNDILD

SEQ ID NO: 9223 - protein, 9 aa, synthetic construct
GGEGTDRLY

SEQ ID NO: 9224 - protein, 9 aa, synthetic construct
GGEGTDRLS

SEQ ID NO: 9225 - protein, 9 aa, synthetic construct
GGRGNDHLD

SEQ ID NO: 9226 - protein, 9 aa, synthetic construct
GGIGDDRLV

SEQ ID NO: 9227 - protein, 9 aa, synthetic construct
GGDGHDLLL

SEQ ID NO: 9228 - protein, 9 aa, synthetic construct
GGLGADRFI

SEQ ID NO: 9229 - protein, 9 aa, synthetic construct
GGAGEDQLT

SEQ ID NO: 9230 - protein, 9 aa, synthetic construct
GGLGADRIE

SEQ ID NO: 9231 - protein, 9 aa, synthetic construct
GGEGNDSIG

SEQ ID NO: 9232 - protein, 9 aa, synthetic construct
GGTGQDTLQ

SEQ ID NO: 9233 - protein, 9 aa, synthetic construct
GGTGQDRLF

SEQ ID NO: 9234 - protein, 9 aa, synthetic construct
GGGGDDWIS

SEQ ID NO: 9235 - protein, 9 aa, synthetic construct
GGDGHDLLV

SEQ ID NO: 9236 - protein, 9 aa, synthetic construct
GGGGADILE

SEQ ID NO: 9237 - protein, 9 aa, synthetic construct
GGRGLDLLI

SEQ ID NO: 9238 - protein, 9 aa, synthetic construct
GGAGRDALA

SEQ ID NO: 9239 - protein, 9 aa, synthetic construct
GGDGDDFLI

SEQ ID NO: 9240 - protein, 9 aa, synthetic construct
GGTGQDTLA

SEQ ID NO: 9241 - protein, 9 aa, synthetic construct
GGLGADRMI

SEQ ID NO: 9242 - protein, 9 aa, synthetic construct
GGDGSDMLF

SEQ ID NO: 9243 - protein, 9 aa, synthetic construct
GGAGEDSLD

SEQ ID NO: 9244 - protein, 9 aa, synthetic construct
GGRGNDKLF

SEQ ID NO: 9245 - protein, 9 aa, synthetic construct
GGIGDDSLS

SEQ ID NO: 9246 - protein, 9 aa, synthetic construct
GGAGEDTIL

SEQ ID NO: 9247 - protein, 9 aa, synthetic construct
GGEGRDKMV

SEQ ID NO: 9248 - protein, 9 aa, synthetic construct
GGTGNDWLQ

SEQ ID NO: 9249 - protein, 9 aa, synthetic construct
GGAGEDTIF

SEQ ID NO: 9250 - protein, 9 aa, synthetic construct
GGAGQDTFI

SEQ ID NO: 9251 - protein, 9 aa, synthetic construct
GGRGNDMLD

SEQ ID NO: 9252 - protein, 9 aa, synthetic construct
GGEGADSLH

SEQ ID NO: 9253 - protein, 9 aa, synthetic construct
GGRGNDLVN

SEQ ID NO: 9254 - protein, 9 aa, synthetic construct
GGEGTDTAS

SEQ ID NO: 9255 - protein, 9 aa, synthetic construct
GGRGNDLLQ

SEQ ID NO: 9256 - protein, 9 aa, synthetic construct
GGRGNDLLL

SEQ ID NO: 9257 - protein, 9 aa, synthetic construct
GGRGNDLLK

SEQ ID NO: 9258 - protein, 9 aa, synthetic construct
GGDGADILF

SEQ ID NO: 9259 - protein, 9 aa, synthetic construct
GGNGTDRLA

SEQ ID NO: 9260 - protein, 9 aa, synthetic construct
GGDGSDLYL

SEQ ID NO: 9261 - protein, 9 aa, synthetic construct
GGAGQDTLA

SEQ ID NO: 9262 - protein, 9 aa, synthetic construct
GGAGQDTLE

SEQ ID NO: 9263 - protein, 9 aa, synthetic construct
GGEGTDTAD

SEQ ID NO: 9264 - protein, 9 aa, synthetic construct
GGDGNDFLG

SEQ ID NO: 9265 - protein, 9 aa, synthetic construct
GGGGADILS

SEQ ID NO: 9266 - protein, 9 aa, synthetic construct
GGIGDDLLN

SEQ ID NO: 9267 - protein, 9 aa, synthetic construct
GGNGADLLL

SEQ ID NO: 9268 - protein, 9 aa, synthetic construct
GGRGGDRLV

SEQ ID NO: 9269 - protein, 9 aa, synthetic construct
GGIGDDILT

SEQ ID NO: 9270 - protein, 9 aa, synthetic construct
GGAGEDILF

SEQ ID NO: 9271 - protein, 9 aa, synthetic construct
GGAGEDILD

SEQ ID NO: 9272 - protein, 9 aa, synthetic construct
GGDGEDTLT

SEQ ID NO: 9273 - protein, 9 aa, synthetic construct
GGDGSDRLD

SEQ ID NO: 9274 - protein, 9 aa, synthetic construct
GGRGGDTLD

SEQ ID NO: 9275 - protein, 9 aa, synthetic construct
GGLGADTLM

SEQ ID NO: 9276 - protein, 9 aa, synthetic construct
GGEGDDYLY

SEQ ID NO: 9277 - protein, 9 aa, synthetic construct
GGEGNDSLW

SEQ ID NO: 9278 - protein, 9 aa, synthetic construct
GGRGGDRLQ

SEQ ID NO: 9279 - protein, 9 aa, synthetic construct
GGAGRDDLD

SEQ ID NO: 9280 - protein, 9 aa, synthetic construct
GGAGRDILL

SEQ ID NO: 9281 - protein, 9 aa, synthetic construct
GGNGVDKLY

SEQ ID NO: 9282 - protein, 9 aa, synthetic construct
GGAGRDILV

SEQ ID NO: 9283 - protein, 9 aa, synthetic construct
GGDGADHID

SEQ ID NO: 9284 - protein, 9 aa, synthetic construct
GGAGADKMY

SEQ ID NO: 9285 - protein, 9 aa, synthetic construct
GGDGSDRLV

SEQ ID NO: 9286 - protein, 9 aa, synthetic construct
GGLGADTMY

SEQ ID NO: 9287 - protein, 9 aa, synthetic construct
GGNGADHME

SEQ ID NO: 9288 - protein, 9 aa, synthetic construct
GGEGDDALG

SEQ ID NO: 9289 - protein, 9 aa, synthetic construct
GGRGHDLIR

SEQ ID NO: 9290 - protein, 9 aa, synthetic construct
GGLGTDTAS

SEQ ID NO: 9291 - protein, 9 aa, synthetic construct
GGDGDDTIA

SEQ ID NO: 9292 - protein, 9 aa, synthetic construct
GGAGRDGLT

SEQ ID NO: 9293 - protein, 9 aa, synthetic construct
GGGGQDTLD

SEQ ID NO: 9294 - protein, 9 aa, synthetic construct
GGLGADSFV

SEQ ID NO: 9295 - protein, 9 aa, synthetic construct
GGAGRDDLT

SEQ ID NO: 9296 - protein, 9 aa, synthetic construct
GGDGHDLLY

SEQ ID NO: 9297 - protein, 9 aa, synthetic construct
GGIGDDLLD

SEQ ID NO: 9298 - protein, 9 aa, synthetic construct
GGNGTDSLY

SEQ ID NO: 9299 - protein, 9 aa, synthetic construct
GGLGADSLA

SEQ ID NO: 9300 - protein, 9 aa, synthetic construct
GGGGQDTLF

SEQ ID NO: 9301 - protein, 9 aa, synthetic construct
GGLGADSLY

SEQ ID NO: 9302 - protein, 9 aa, synthetic construct
GGNGTDTLN

SEQ ID NO: 9303 - protein, 9 aa, synthetic construct
GGTGRDAFV

SEQ ID NO: 9304 - protein, 9 aa, synthetic construct
GGLGADSMV

SEQ ID NO: 9305 - protein, 9 aa, synthetic construct
GGDGDDFIV

SEQ ID NO: 9306 - protein, 9 aa, synthetic construct
GGAGEDLFV

SEQ ID NO: 9307 - protein, 9 aa, synthetic construct
GGLGNDRMD

SEQ ID NO: 9308 - protein, 9 aa, synthetic construct
GGAGADKLW

SEQ ID NO: 9309 - protein, 9 aa, synthetic construct
GGRGHDTLY

SEQ ID NO: 9310 - protein, 9 aa, synthetic construct
GGLGNDRLQ

SEQ ID NO: 9311 - protein, 9 aa, synthetic construct
GGGGADKLT

SEQ ID NO: 9312 - protein, 9 aa, synthetic construct
GGRGNDNLS

SEQ ID NO: 9313 - protein, 9 aa, synthetic construct
GGTGNDWIS

SEQ ID NO: 9314 - protein, 9 aa, synthetic construct
GGEGHDTLD

SEQ ID NO: 9315 - protein, 9 aa, synthetic construct
GGTGNDRMF

SEQ ID NO: 9316 - protein, 9 aa, synthetic construct
GGGGGDSLF

SEQ ID NO: 9317 - protein, 9 aa, synthetic construct
GGAGEDWLL

SEQ ID NO: 9318 - protein, 9 aa, synthetic construct
GGSGADLLE

SEQ ID NO: 9319 - protein, 9 aa, synthetic construct
GGAGADIVT

SEQ ID NO: 9320 - protein, 9 aa, synthetic construct
GGTGNDRII

SEQ ID NO: 9321 - protein, 9 aa, synthetic construct
GGAGADIYI

SEQ ID NO: 9322 - protein, 9 aa, synthetic construct
GGDGNDHID

SEQ ID NO: 9323 - protein, 9 aa, synthetic construct
GGDGGDNLD

SEQ ID NO: 9324 - protein, 9 aa, synthetic construct
GGTGNDRMA

SEQ ID NO: 9325 - protein, 9 aa, synthetic construct
GGEGHDRLY

SEQ ID NO: 9326 - protein, 9 aa, synthetic construct
GGLGADIFL

SEQ ID NO: 9327 - protein, 9 aa, synthetic construct
GGGGNDLIF

SEQ ID NO: 9328 - protein, 9 aa, synthetic construct
GGEGTDVLT

SEQ ID NO: 9329 - protein, 9 aa, synthetic construct
GGGGTDILN

SEQ ID NO: 9330 - protein, 9 aa, synthetic construct
GGEGNDRLR

SEQ ID NO: 9331 - protein, 9 aa, synthetic construct
GGDGADKLN

SEQ ID NO: 9332 - protein, 9 aa, synthetic construct
GGIGDDVFV

SEQ ID NO: 9333 - protein, 9 aa, synthetic construct
GGRGQDILS

SEQ ID NO: 9334 - protein, 9 aa, synthetic construct
GGAGQDLLQ

SEQ ID NO: 9335 - protein, 9 aa, synthetic construct
GGEGNDRLT

SEQ ID NO: 9336 - protein, 9 aa, synthetic construct
GGGGADDFT

SEQ ID NO: 9337 - protein, 9 aa, synthetic construct
GGAGQDHLM

SEQ ID NO: 9338 - protein, 9 aa, synthetic construct
GGLGADALT

SEQ ID NO: 9339 - protein, 9 aa, synthetic construct
GGGGADCFV

SEQ ID NO: 9340 - protein, 9 aa, synthetic construct
GGEGDDQLD

SEQ ID NO: 9341 - protein, 9 aa, synthetic construct
GGIGDDWLD

SEQ ID NO: 9342 - protein, 9 aa, synthetic construct
GGKGWDRII

SEQ ID NO: 9343 - protein, 9 aa, synthetic construct
GGTGNDNLN

SEQ ID NO: 9344 - protein, 9 aa, synthetic construct
GGNGSDTIY

SEQ ID NO: 9345 - protein, 9 aa, synthetic construct
GGEGNDRLC

SEQ ID NO: 9346 - protein, 9 aa, synthetic construct
GGNGSDTLE

SEQ ID NO: 9347 - protein, 9 aa, synthetic construct
GGNGSDTLF

SEQ ID NO: 9348 - protein, 9 aa, synthetic construct
GGDGDDHLA

SEQ ID NO: 9349 - protein, 9 aa, synthetic construct
GGAGQDEIN

SEQ ID NO: 9350 - protein, 9 aa, synthetic construct
GGGGNDLIS

SEQ ID NO: 9351 - protein, 9 aa, synthetic construct
GGTGNDQIY

SEQ ID NO: 9352 - protein, 9 aa, synthetic construct
GGNGSDTLY

SEQ ID NO: 9353 - protein, 9 aa, synthetic construct
GGLGNDSLQ

SEQ ID NO: 9354 - protein, 9 aa, synthetic construct
GGTGNDQLT

SEQ ID NO: 9355 - protein, 9 aa, synthetic construct
GGTGNDQLW

SEQ ID NO: 9356 - protein, 9 aa, synthetic construct
GGNGGDSVL

SEQ ID NO: 9357 - protein, 9 aa, synthetic construct
GGIGDDVLR

SEQ ID NO: 9358 - protein, 9 aa, synthetic construct
GGLGNDSLK

SEQ ID NO: 9359 - protein, 9 aa, synthetic construct
GGEGNDRLW

SEQ ID NO: 9360 - protein, 9 aa, synthetic construct
GGGGADELV

SEQ ID NO: 9361 - protein, 9 aa, synthetic construct
GGGGADHFI

SEQ ID NO: 9362 - protein, 9 aa, synthetic construct
GGTGNDVLW

SEQ ID NO: 9363 - protein, 9 aa, synthetic construct
GGTGNDTVA

SEQ ID NO: 9364 - protein, 9 aa, synthetic construct
GGRGNDTIN

SEQ ID NO: 9365 - protein, 9 aa, synthetic construct
GGNGSDVLQ

SEQ ID NO: 9366 - protein, 9 aa, synthetic construct
GGIGDDTLT

SEQ ID NO: 9367 - protein, 9 aa, synthetic construct
GGTGNDVFT

SEQ ID NO: 9368 - protein, 9 aa, synthetic construct
GGNGSDYID

SEQ ID NO: 9369 - protein, 9 aa, synthetic construct
GGRGNDSLY

SEQ ID NO: 9370 - protein, 9 aa, synthetic construct
GGRGNDSLA

SEQ ID NO: 9371 - protein, 9 aa, synthetic construct
GGNGSDYLL

SEQ ID NO: 9372 - protein, 9 aa, synthetic construct
GGAGEDTLQ

SEQ ID NO: 9373 - protein, 9 aa, synthetic construct
GGGGTDILR

SEQ ID NO: 9374 - protein, 9 aa, synthetic construct
GGNGTDFLN

SEQ ID NO: 9375 - protein, 9 aa, synthetic construct
GGAGEDTLK

SEQ ID NO: 9376 - protein, 9 aa, synthetic construct
GGIGDDTLA

SEQ ID NO: 9377 - protein, 9 aa, synthetic construct
GGGGDDWLF

SEQ ID NO: 9378 - protein, 9 aa, synthetic construct
GGDGSDLLW

SEQ ID NO: 9379 - protein, 9 aa, synthetic construct
GGGGDDWLE

SEQ ID NO: 9380 - protein, 9 aa, synthetic construct
GGAGQDSLS

SEQ ID NO: 9381 - protein, 9 aa, synthetic construct
GGRGNDQLI

SEQ ID NO: 9382 - protein, 9 aa, synthetic construct
GGIGDDTIF

SEQ ID NO: 9383 - protein, 9 aa, synthetic construct
GGTGNDTIQ

SEQ ID NO: 9384 - protein, 9 aa, synthetic construct
GGTGNDTIG

SEQ ID NO: 9385 - protein, 9 aa, synthetic construct
GGGGGDSLL

SEQ ID NO: 9386 - protein, 9 aa, synthetic construct
GGDGSDLLL

SEQ ID NO: 9387 - protein, 9 aa, synthetic construct
GGAGEDVLT

SEQ ID NO: 9388 - protein, 9 aa, synthetic construct
GGDGYDTIN

SEQ ID NO: 9389 - protein, 9 aa, synthetic construct
GGLGADILN

SEQ ID NO: 9390 - protein, 9 aa, synthetic construct
GGLGADILS

SEQ ID NO: 9391 - protein, 9 aa, synthetic construct
GGMGDDLLD

SEQ ID NO: 9392 - protein, 9 aa, synthetic construct
GGEGHDQAV

SEQ ID NO: 9393 - protein, 9 aa, synthetic construct
GGRGNDVVL

SEQ ID NO: 9394 - protein, 9 aa, synthetic construct
GGRGNDVMR

SEQ ID NO: 9395 - protein, 9 aa, synthetic construct
GGGGGDALF

SEQ ID NO: 9396 - protein, 9 aa, synthetic construct
GGDGADKLD

SEQ ID NO: 9397 - protein, 9 aa, synthetic construct
GGEGDDYLE

SEQ ID NO: 9398 - protein, 9 aa, synthetic construct
GGRGNDVLK

SEQ ID NO: 9399 - protein, 9 aa, synthetic construct
GGLGRDTLV

SEQ ID NO: 9400 - protein, 9 aa, synthetic construct
GGRGNDVIR

SEQ ID NO: 9401 - protein, 9 aa, synthetic construct
GGRGNDTYM

SEQ ID NO: 9402 - protein, 9 aa, synthetic construct
GGEGDDTYN

SEQ ID NO: 9403 - protein, 9 aa, synthetic construct
GGRGNDTVL

SEQ ID NO: 9404 - protein, 9 aa, synthetic construct
GGEGTDTLV

SEQ ID NO: 9405 - protein, 9 aa, synthetic construct
GGNGSDVLN

SEQ ID NO: 9406 - protein, 9 aa, synthetic construct
GGGGADDFV

SEQ ID NO: 9407 - protein, 9 aa, synthetic construct
GGSGADRMA

SEQ ID NO: 9408 - protein, 9 aa, synthetic construct
GGSGADLLH

SEQ ID NO: 9409 - protein, 9 aa, synthetic construct
GGTGDDTLC

SEQ ID NO: 9410 - protein, 9 aa, synthetic construct
GGAGADDFI

SEQ ID NO: 9411 - protein, 9 aa, synthetic construct
GGTGDDTMT

SEQ ID NO: 9412 - protein, 9 aa, synthetic construct
GGSGDDTYF

SEQ ID NO: 9413 - protein, 9 aa, synthetic construct
GGSGDDTVT

SEQ ID NO: 9414 - protein, 9 aa, synthetic construct
GGKGNDTLM

SEQ ID NO: 9415 - protein, 9 aa, synthetic construct
GGTGDDVFI

SEQ ID NO: 9416 - protein, 9 aa, synthetic construct
GGTGDDVFR

SEQ ID NO: 9417 - protein, 9 aa, synthetic construct
GGIGNDTYN

SEQ ID NO: 9418 - protein, 9 aa, synthetic construct
GGAGNDQMD

SEQ ID NO: 9419 - protein, 9 aa, synthetic construct
GGTGDDVIT

SEQ ID NO: 9420 - protein, 9 aa, synthetic construct
GGSGDDTLM

SEQ ID NO: 9421 - protein, 9 aa, synthetic construct
GGTGDDVLM

SEQ ID NO: 9422 - protein, 9 aa, synthetic construct
GGDGDDRFD

SEQ ID NO: 9423 - protein, 9 aa, synthetic construct
GGAGHDILT

SEQ ID NO: 9424 - protein, 9 aa, synthetic construct
GGDGRDLLF

SEQ ID NO: 9425 - protein, 9 aa, synthetic construct
GGIGNDTVS

SEQ ID NO: 9426 - protein, 9 aa, synthetic construct
GGDGRDLLI

SEQ ID NO: 9427 - protein, 9 aa, synthetic construct
GGNGNDVIT

SEQ ID NO: 9428 - protein, 9 aa, synthetic construct
GGIGNDTMI

SEQ ID NO: 9429 - protein, 9 aa, synthetic construct
GGNGDDALD

SEQ ID NO: 9430 - protein, 9 aa, synthetic construct
GGEGQDTLD

SEQ ID NO: 9431 - protein, 9 aa, synthetic construct
GGKGNDTIN

SEQ ID NO: 9432 - protein, 9 aa, synthetic construct
GGTGDDTIH

SEQ ID NO: 9433 - protein, 9 aa, synthetic construct
GGTGDDSLE

SEQ ID NO: 9434 - protein, 9 aa, synthetic construct
GGSGDDVVA

SEQ ID NO: 9435 - protein, 9 aa, synthetic construct
GGSGDDVML

SEQ ID NO: 9436 - protein, 9 aa, synthetic construct
GGIGNDVLR

SEQ ID NO: 9437 - protein, 9 aa, synthetic construct
GGTGDDSLW

SEQ ID NO: 9438 - protein, 9 aa, synthetic construct
GGNGNDTVS

SEQ ID NO: 9439 - protein, 9 aa, synthetic construct
GGNGNDTVT

SEQ ID NO: 9440 - protein, 9 aa, synthetic construct
GGIGNDVLL

SEQ ID NO: 9441 - protein, 9 aa, synthetic construct
GGTGDDSVA

SEQ ID NO: 9442 - protein, 9 aa, synthetic construct
GGIGNDVLH

SEQ ID NO: 9443 - protein, 9 aa, synthetic construct
GGNGNDTVY

SEQ ID NO: 9444 - protein, 9 aa, synthetic construct
GGIGNDVLE

SEQ ID NO: 9445 - protein, 9 aa, synthetic construct
GGIGNDVLA

SEQ ID NO: 9446 - protein, 9 aa, synthetic construct
GGTGDDTFL

SEQ ID NO: 9447 - protein, 9 aa, synthetic construct
GGSGDDVIH

SEQ ID NO: 9448 - protein, 9 aa, synthetic construct
GGIGNDVID

SEQ ID NO: 9449 - protein, 9 aa, synthetic construct
GGDGADTVI

SEQ ID NO: 9450 - protein, 9 aa, synthetic construct
GGTGDDTIG

SEQ ID NO: 9451 - protein, 9 aa, synthetic construct
GGSGDDVFV

SEQ ID NO: 9452 - protein, 9 aa, synthetic construct
GGAGNDQMR

SEQ ID NO: 9453 - protein, 9 aa, synthetic construct
GGAGADDLA

SEQ ID NO: 9454 - protein, 9 aa, synthetic construct
GGIGNDTLK

SEQ ID NO: 9455 - protein, 9 aa, synthetic construct
GGTGDDYLN

SEQ ID NO: 9456 - protein, 9 aa, synthetic construct
GGTGEDTFI

SEQ ID NO: 9457 - protein, 9 aa, synthetic construct
GGAGNDRIH

SEQ ID NO: 9458 - protein, 9 aa, synthetic construct
GGSGDDQLL

SEQ ID NO: 9459 - protein, 9 aa, synthetic construct
GGDGADTFF

SEQ ID NO: 9460 - protein, 9 aa, synthetic construct
GGKGNDVLR

SEQ ID NO: 9461 - protein, 9 aa, synthetic construct
GGKGNDVLS

SEQ ID NO: 9462 - protein, 9 aa, synthetic construct
GGLGNDVVN

SEQ ID NO: 9463 - protein, 9 aa, synthetic construct
GGGGSDLII

SEQ ID NO: 9464 - protein, 9 aa, synthetic construct
GGGGSDTFA

SEQ ID NO: 9465 - protein, 9 aa, synthetic construct
GGYGNDYLN

SEQ ID NO: 9466 - protein, 9 aa, synthetic construct
GGAGGDWLD

SEQ ID NO: 9467 - protein, 9 aa, synthetic construct
GGFGADRLF

SEQ ID NO: 9468 - protein, 9 aa, synthetic construct
GGFGADRLE

SEQ ID NO: 9469 - protein, 9 aa, synthetic construct
GGTGFDLLK

SEQ ID NO: 9470 - protein, 9 aa, synthetic construct
GGKGNDVLY

SEQ ID NO: 9471 - protein, 9 aa, synthetic construct
GGDGDDRIT

SEQ ID NO: 9472 - protein, 9 aa, synthetic construct
GGYGNDYLF

SEQ ID NO: 9473 - protein, 9 aa, synthetic construct
GGGGNDVMT

SEQ ID NO: 9474 - protein, 9 aa, synthetic construct
GGDGADSYV

SEQ ID NO: 9475 - protein, 9 aa, synthetic construct
GGKGNDVLE

SEQ ID NO: 9476 - protein, 9 aa, synthetic construct
GGSGDDRMF

SEQ ID NO: 9477 - protein, 9 aa, synthetic construct
GGAGHDDLY

SEQ ID NO: 9478 - protein, 9 aa, synthetic construct
GGKGNDTYL

SEQ ID NO: 9479 - protein, 9 aa, synthetic construct
GGAGNDQVF

SEQ ID NO: 9480 - protein, 9 aa, synthetic construct
GGYGRDTMS

SEQ ID NO: 9481 - protein, 9 aa, synthetic construct
GGIGNDTIW

SEQ ID NO: 9482 - protein, 9 aa, synthetic construct
GGIGNDTIT

SEQ ID NO: 9483 - protein, 9 aa, synthetic construct
GGIGNDTIS

SEQ ID NO: 9484 - protein, 9 aa, synthetic construct
GGAGHDFLQ

SEQ ID NO: 9485 - protein, 9 aa, synthetic construct
GGKGNDTYK

SEQ ID NO: 9486 - protein, 9 aa, synthetic construct
GGSGDDSLG

SEQ ID NO: 9487 - protein, 9 aa, synthetic construct
GGAGADDMD

SEQ ID NO: 9488 - protein, 9 aa, synthetic construct
GGKGNDVLA

SEQ ID NO: 9489 - protein, 9 aa, synthetic construct
GGMGADTLR

SEQ ID NO: 9490 - protein, 9 aa, synthetic construct
GGAGNDQVL

SEQ ID NO: 9491 - protein, 9 aa, synthetic construct
GGAGADDMR

SEQ ID NO: 9492 - protein, 9 aa, synthetic construct
GGIGNDTIA

SEQ ID NO: 9493 - protein, 9 aa, synthetic construct
GGKGNDVID

SEQ ID NO: 9494 - protein, 9 aa, synthetic construct
GGDGRDLLV

SEQ ID NO: 9495 - protein, 9 aa, synthetic construct
GGTGEDLLN

SEQ ID NO: 9496 - protein, 9 aa, synthetic construct
GGDGDDIVS

SEQ ID NO: 9497 - protein, 9 aa, synthetic construct
GGKGNDTIY

SEQ ID NO: 9498 - protein, 9 aa, synthetic construct
GGIGNDVLT

SEQ ID NO: 9499 - protein, 9 aa, synthetic construct
GGDGNDLIG

SEQ ID NO: 9500 - protein, 9 aa, synthetic construct
GGAGNDLMV

SEQ ID NO: 9501 - protein, 9 aa, synthetic construct
GGAGNDLVL

SEQ ID NO: 9502 - protein, 9 aa, synthetic construct
GGKGNDLLY

SEQ ID NO: 9503 - protein, 9 aa, synthetic construct
GGTGDDLIH

SEQ ID NO: 9504 - protein, 9 aa, synthetic construct
GGDGRDILN

SEQ ID NO: 9505 - protein, 9 aa, synthetic construct
GGAGNDLVY

SEQ ID NO: 9506 - protein, 9 aa, synthetic construct
GGDGNDQLK

SEQ ID NO: 9507 - protein, 9 aa, synthetic construct
GGTGDDLLH

SEQ ID NO: 9508 - protein, 9 aa, synthetic construct
GGAGADAIT

SEQ ID NO: 9509 - protein, 9 aa, synthetic construct
GGDGNDQLH

SEQ ID NO: 9510 - protein, 9 aa, synthetic construct
GGNGNDTIL

SEQ ID NO: 9511 - protein, 9 aa, synthetic construct
GGAGHDRID

SEQ ID NO: 9512 - protein, 9 aa, synthetic construct
GGAGNDMFV

SEQ ID NO: 9513 - protein, 9 aa, synthetic construct
GGAGADALK

SEQ ID NO: 9514 - protein, 9 aa, synthetic construct
GGAGNDMID

SEQ ID NO: 9515 - protein, 9 aa, synthetic construct
GGEGNDIIY

SEQ ID NO: 9516 - protein, 9 aa, synthetic construct
GGKGNDNLS

SEQ ID NO: 9517 - protein, 9 aa, synthetic construct
GGGGGDRLE

SEQ ID NO: 9518 - protein, 9 aa, synthetic construct
GGTGDDLYI

SEQ ID NO: 9519 - protein, 9 aa, synthetic construct
GGTGDDLYL

SEQ ID NO: 9520 - protein, 9 aa, synthetic construct
GGAGADAIR

SEQ ID NO: 9521 - protein, 9 aa, synthetic construct
GGTGDDLFI

SEQ ID NO: 9522 - protein, 9 aa, synthetic construct
GGIGNDVLV

SEQ ID NO: 9523 - protein, 9 aa, synthetic construct
GGEGDDRLI

SEQ ID NO: 9524 - protein, 9 aa, synthetic construct
GGEGADTME

SEQ ID NO: 9525 - protein, 9 aa, synthetic construct
GGTGDDIFH

SEQ ID NO: 9526 - protein, 9 aa, synthetic construct
GGEGNDIIK

SEQ ID NO: 9527 - protein, 9 aa, synthetic construct
GGTGDDIIT

SEQ ID NO: 9528 - protein, 9 aa, synthetic construct
GGAGADAAW

SEQ ID NO: 9529 - protein, 9 aa, synthetic construct
GGSGFDYLV

SEQ ID NO: 9530 - protein, 9 aa, synthetic construct
GGTGDDILA

SEQ ID NO: 9531 - protein, 9 aa, synthetic construct
GGIGQDTFQ

SEQ ID NO: 9532 - protein, 9 aa, synthetic construct
GGDGEDTAD

SEQ ID NO: 9533 - protein, 9 aa, synthetic construct
GGSGFDVLE

SEQ ID NO: 9534 - protein, 9 aa, synthetic construct
GGTGDDIVI

SEQ ID NO: 9535 - protein, 9 aa, synthetic construct
GGAGHDRLV

SEQ ID NO: 9536 - protein, 9 aa, synthetic construct
GGGGHDHLD

SEQ ID NO: 9537 - protein, 9 aa, synthetic construct
GGAGHDRLT

SEQ ID NO: 9538 - protein, 9 aa, synthetic construct
GGTGDDKLH

SEQ ID NO: 9539 - protein, 9 aa, synthetic construct
GGTGDDKLI

SEQ ID NO: 9540 - protein, 9 aa, synthetic construct
GGAGNDLMK

SEQ ID NO: 9541 - protein, 9 aa, synthetic construct
GGAGADAIF

SEQ ID NO: 9542 - protein, 9 aa, synthetic construct
GGAGNDLMN

SEQ ID NO: 9543 - protein, 9 aa, synthetic construct
GGFGRDTLT

SEQ ID NO: 9544 - protein, 9 aa, synthetic construct
GGTGDDLYY

SEQ ID NO: 9545 - protein, 9 aa, synthetic construct
GGDGRDIVY

SEQ ID NO: 9546 - protein, 9 aa, synthetic construct
GGIGNDYLS

SEQ ID NO: 9547 - protein, 9 aa, synthetic construct
GGTGDDRIH

SEQ ID NO: 9548 - protein, 9 aa, synthetic construct
GGAGNDNLW

SEQ ID NO: 9549 - protein, 9 aa, synthetic construct
GGEGADTLV

SEQ ID NO: 9550 - protein, 9 aa, synthetic construct
GGGGNDNLF

SEQ ID NO: 9551 - protein, 9 aa, synthetic construct
GGAGHDLLS

SEQ ID NO: 9552 - protein, 9 aa, synthetic construct
GGAGHDLLR

SEQ ID NO: 9553 - protein, 9 aa, synthetic construct
GGDGADTVF

SEQ ID NO: 9554 - protein, 9 aa, synthetic construct
GGGGSDLLV

SEQ ID NO: 9555 - protein, 9 aa, synthetic construct
GGKGNDSYF

SEQ ID NO: 9556 - protein, 9 aa, synthetic construct
GGEGADFLG

SEQ ID NO: 9557 - protein, 9 aa, synthetic construct
GGDGNDNLT

SEQ ID NO: 9558 - protein, 9 aa, synthetic construct
GGEGQDQIH

SEQ ID NO: 9559 - protein, 9 aa, synthetic construct
GGGGSDRLS

SEQ ID NO: 9560 - protein, 9 aa, synthetic construct
GGAGNDPLR

SEQ ID NO: 9561 - protein, 9 aa, synthetic construct
GGTGDDRMY

SEQ ID NO: 9562 - protein, 9 aa, synthetic construct
GGEGQDTFV

SEQ ID NO: 9563 - protein, 9 aa, synthetic construct
GGDGNDNLK

SEQ ID NO: 9564 - protein, 9 aa, synthetic construct
GGAGHDLLI

SEQ ID NO: 9565 - protein, 9 aa, synthetic construct
GGLGSDTVV

SEQ ID NO: 9566 - protein, 9 aa, synthetic construct
GGSGEDDYD

SEQ ID NO: 9567 - protein, 9 aa, synthetic construct
GGTGDDRIF

SEQ ID NO: 9568 - protein, 9 aa, synthetic construct
GGNGNDTLM

SEQ ID NO: 9569 - protein, 9 aa, synthetic construct
GGSGEDLLL

SEQ ID NO: 9570 - protein, 9 aa, synthetic construct
GGYGTDFLN

SEQ ID NO: 9571 - protein, 9 aa, synthetic construct
GGGGNDVIF

SEQ ID NO: 9572 - protein, 9 aa, synthetic construct
GGSGEDRLR

SEQ ID NO: 9573 - protein, 9 aa, synthetic construct
GGEGADFLR

SEQ ID NO: 9574 - protein, 9 aa, synthetic construct
GGTGDDNLS

SEQ ID NO: 9575 - protein, 9 aa, synthetic construct
GGAGNDMVD

SEQ ID NO: 9576 - protein, 9 aa, synthetic construct
GGAGHDMLS

SEQ ID NO: 9577 - protein, 9 aa, synthetic construct
GGDGNDQIA

SEQ ID NO: 9578 - protein, 9 aa, synthetic construct
GGIGNDWLD

SEQ ID NO: 9579 - protein, 9 aa, synthetic construct
GGTGDDRIA

SEQ ID NO: 9580 - protein, 9 aa, synthetic construct
GGTGDDQLH

SEQ ID NO: 9581 - protein, 9 aa, synthetic construct
GGAGNDNIR

SEQ ID NO: 9582 - protein, 9 aa, synthetic construct
GGAGNDNIS

SEQ ID NO: 9583 - protein, 9 aa, synthetic construct
GGNGEDLLT

SEQ ID NO: 9584 - protein, 9 aa, synthetic construct
GGEGNDILQ

SEQ ID NO: 9585 - protein, 9 aa, synthetic construct
GGAGNDNLA

SEQ ID NO: 9586 - protein, 9 aa, synthetic construct
GGIGNDVYV

SEQ ID NO: 9587 - protein, 9 aa, synthetic construct
GGAGNDNLE

SEQ ID NO: 9588 - protein, 9 aa, synthetic construct
GGDGRDQID

SEQ ID NO: 9589 - protein, 9 aa, synthetic construct
GGGGSDTFF

SEQ ID NO: 9590 - protein, 9 aa, synthetic construct
GGAGNDRMD

SEQ ID NO: 9591 - protein, 9 aa, synthetic construct
GGSGADTMV

SEQ ID NO: 9592 - protein, 9 aa, synthetic construct
GGSGADTMQ

SEQ ID NO: 9593 - protein, 9 aa, synthetic construct
GGSGADTML

SEQ ID NO: 9594 - protein, 9 aa, synthetic construct
GGGGHDTLW

SEQ ID NO: 9595 - protein, 9 aa, synthetic construct
GGSGADTMD

SEQ ID NO: 9596 - protein, 9 aa, synthetic construct
GGSGADTLW

SEQ ID NO: 9597 - protein, 9 aa, synthetic construct
GGTGIDTLL

SEQ ID NO: 9598 - protein, 9 aa, synthetic construct
GGYGNDILQ

SEQ ID NO: 9599 - protein, 9 aa, synthetic construct
GGAGGDILI

SEQ ID NO: 9600 - protein, 9 aa, synthetic construct
GGTGIDTML

SEQ ID NO: 9601 - protein, 9 aa, synthetic construct
GGTGIDTVV

SEQ ID NO: 9602 - protein, 9 aa, synthetic construct
GGGGNDYIN

SEQ ID NO: 9603 - protein, 9 aa, synthetic construct
GGNGRDTIS

SEQ ID NO: 9604 - protein, 9 aa, synthetic construct
GGDGRDTLV

SEQ ID NO: 9605 - protein, 9 aa, synthetic construct
GGNGRDTIY

SEQ ID NO: 9606 - protein, 9 aa, synthetic construct
GGSGADTAV

SEQ ID NO: 9607 - protein, 9 aa, synthetic construct
GGSGADTAT

SEQ ID NO: 9608 - protein, 9 aa, synthetic construct
GGIGNDAYY

SEQ ID NO: 9609 - protein, 9 aa, synthetic construct
GGSGADSMV

SEQ ID NO: 9610 - protein, 9 aa, synthetic construct
GGDGADQLL

SEQ ID NO: 9611 - protein, 9 aa, synthetic construct
GGTGIDSLT

SEQ ID NO: 9612 - protein, 9 aa, synthetic construct
GGDGADQLY

SEQ ID NO: 9613 - protein, 9 aa, synthetic construct
GGLGNDVMI

SEQ ID NO: 9614 - protein, 9 aa, synthetic construct
GGNGRDSMW

SEQ ID NO: 9615 - protein, 9 aa, synthetic construct
GGNGFDILV

SEQ ID NO: 9616 - protein, 9 aa, synthetic construct
GGIGNDILF

SEQ ID NO: 9617 - protein, 9 aa, synthetic construct
GGSGADVMQ

SEQ ID NO: 9618 - protein, 9 aa, synthetic construct
GGLGNDTVN

SEQ ID NO: 9619 - protein, 9 aa, synthetic construct
GGDGDDRMS

SEQ ID NO: 9620 - protein, 9 aa, synthetic construct
GGYGNDLIY

SEQ ID NO: 9621 - protein, 9 aa, synthetic construct
GGSGADVLQ

SEQ ID NO: 9622 - protein, 9 aa, synthetic construct
GGAGGDLLF

SEQ ID NO: 9623 - protein, 9 aa, synthetic construct
GGAGGDLLE

SEQ ID NO: 9624 - protein, 9 aa, synthetic construct
GGGGSDTYR

SEQ ID NO: 9625 - protein, 9 aa, synthetic construct
GGAGGDLIR

SEQ ID NO: 9626 - protein, 9 aa, synthetic construct
GGDGNDLMI

SEQ ID NO: 9627 - protein, 9 aa, synthetic construct
GGEGADIFR

SEQ ID NO: 9628 - protein, 9 aa, synthetic construct
GGSGADVIT

SEQ ID NO: 9629 - protein, 9 aa, synthetic construct
GGYGNDIYH

SEQ ID NO: 9630 - protein, 9 aa, synthetic construct
GGDGNDLMD

SEQ ID NO: 9631 - protein, 9 aa, synthetic construct
GGAGGDLFV

SEQ ID NO: 9632 - protein, 9 aa, synthetic construct
GGSGADVFA

SEQ ID NO: 9633 - protein, 9 aa, synthetic construct
GGSGADTYQ

SEQ ID NO: 9634 - protein, 9 aa, synthetic construct
GGDGEDRLL

SEQ ID NO: 9635 - protein, 9 aa, synthetic construct
GGSGADSMA

SEQ ID NO: 9636 - protein, 9 aa, synthetic construct
GGAGGDFID

SEQ ID NO: 9637 - protein, 9 aa, synthetic construct
GGIGNDALY

SEQ ID NO: 9638 - protein, 9 aa, synthetic construct
GGSGADQLY

SEQ ID NO: 9639 - protein, 9 aa, synthetic construct
GGAGFDYLN

SEQ ID NO: 9640 - protein, 9 aa, synthetic construct
GGSGADQLS

SEQ ID NO: 9641 - protein, 9 aa, synthetic construct
GGIGKDTLQ

SEQ ID NO: 9642 - protein, 9 aa, synthetic construct
GGTGLDIID

SEQ ID NO: 9643 - protein, 9 aa, synthetic construct
GGAGNDTYQ

SEQ ID NO: 9644 - protein, 9 aa, synthetic construct
GGAGFDWAS

SEQ ID NO: 9645 - protein, 9 aa, synthetic construct
GGEGDDWVV

SEQ ID NO: 9646 - protein, 9 aa, synthetic construct
GGSGADNLH

SEQ ID NO: 9647 - protein, 9 aa, synthetic construct
GGDGADQIG

SEQ ID NO: 9648 - protein, 9 aa, synthetic construct
GGAGNDVAL

SEQ ID NO: 9649 - protein, 9 aa, synthetic construct
GGSGADMLN

SEQ ID NO: 9650 - protein, 9 aa, synthetic construct
GGAGADHLN

SEQ ID NO: 9651 - protein, 9 aa, synthetic construct
GGAGNDVFK

SEQ ID NO: 9652 - protein, 9 aa, synthetic construct
GGDGDDSIA

SEQ ID NO: 9653 - protein, 9 aa, synthetic construct
GGEGRDILF

SEQ ID NO: 9654 - protein, 9 aa, synthetic construct
GGDGADNLY

SEQ ID NO: 9655 - protein, 9 aa, synthetic construct
GGSGADLML

SEQ ID NO: 9656 - protein, 9 aa, synthetic construct
GGNGADSLN

SEQ ID NO: 9657 - protein, 9 aa, synthetic construct
GGAGNDTYG

SEQ ID NO: 9658 - protein, 9 aa, synthetic construct
GGSGADQMT

SEQ ID NO: 9659 - protein, 9 aa, synthetic construct
GGTGKDVLY

SEQ ID NO: 9660 - protein, 9 aa, synthetic construct
GGSGADRMI

SEQ ID NO: 9661 - protein, 9 aa, synthetic construct
GGIGNDALS

SEQ ID NO: 9662 - protein, 9 aa, synthetic construct
GGIGNDALD

SEQ ID NO: 9663 - protein, 9 aa, synthetic construct
GGDGNDLLM

SEQ ID NO: 9664 - protein, 9 aa, synthetic construct
GGSGADSID

SEQ ID NO: 9665 - protein, 9 aa, synthetic construct
GGDGDDILH

SEQ ID NO: 9666 - protein, 9 aa, synthetic construct
GGNGRDTLY

SEQ ID NO: 9667 - protein, 9 aa, synthetic construct
GGNGADTLH

SEQ ID NO: 9668 - protein, 9 aa, synthetic construct
GGEGNDNID

SEQ ID NO: 9669 - protein, 9 aa, synthetic construct
GGDGADGLD

SEQ ID NO: 9670 - protein, 9 aa, synthetic construct
GGSGADRFE

SEQ ID NO: 9671 - protein, 9 aa, synthetic construct
GGDGFDTAD

SEQ ID NO: 9672 - protein, 9 aa, synthetic construct
GGDGRDVLD

SEQ ID NO: 9673 - protein, 9 aa, synthetic construct
GGNGRDVLD

SEQ ID NO: 9674 - protein, 9 aa, synthetic construct
GGSGADRLA

SEQ ID NO: 9675 - protein, 9 aa, synthetic construct
GGGGNDYLN

SEQ ID NO: 9676 - protein, 9 aa, synthetic construct
GGDGRDVLI

SEQ ID NO: 9677 - protein, 9 aa, synthetic construct
GGSGADRFY

SEQ ID NO: 9678 - protein, 9 aa, synthetic construct
GGLGSDWVR

SEQ ID NO: 9679 - protein, 9 aa, synthetic construct
GGDGADTVS

SEQ ID NO: 9680 - protein, 9 aa, synthetic construct
GGGGSDTYH

SEQ ID NO: 9681 - protein, 9 aa, synthetic construct
GGAGNDTFE

SEQ ID NO: 9682 - protein, 9 aa, synthetic construct
GGSGDDHLD

SEQ ID NO: 9683 - protein, 9 aa, synthetic construct
GGFGSDTAA

SEQ ID NO: 9684 - protein, 9 aa, synthetic construct
GGDGADSLE

SEQ ID NO: 9685 - protein, 9 aa, synthetic construct
GGYGNDTLT

SEQ ID NO: 9686 - protein, 9 aa, synthetic construct
GGYGNDTLK

SEQ ID NO: 9687 - protein, 9 aa, synthetic construct
GGAGGDTLH

SEQ ID NO: 9688 - protein, 9 aa, synthetic construct
GGDGRDRIS

SEQ ID NO: 9689 - protein, 9 aa, synthetic construct
GGKGNDYLS

SEQ ID NO: 9690 - protein, 9 aa, synthetic construct
GGIGNDQLF

SEQ ID NO: 9691 - protein, 9 aa, synthetic construct
GGSGDDIVN

SEQ ID NO: 9692 - protein, 9 aa, synthetic construct
GGLGNDVIR

SEQ ID NO: 9693 - protein, 9 aa, synthetic construct
GGTGGDQLS

SEQ ID NO: 9694 - protein, 9 aa, synthetic construct
GGNGQDTLI

SEQ ID NO: 9695 - protein, 9 aa, synthetic construct
GGDGRDRLL

SEQ ID NO: 9696 - protein, 9 aa, synthetic construct
GGTGGDTFK

SEQ ID NO: 9697 - protein, 9 aa, synthetic construct
GGKGQDEIK

SEQ ID NO: 9698 - protein, 9 aa, synthetic construct
GGEGRDCLD

SEQ ID NO: 9699 - protein, 9 aa, synthetic construct
GGAGGDTFI

SEQ ID NO: 9700 - protein, 9 aa, synthetic construct
GGGGGDILF

SEQ ID NO: 9701 - protein, 9 aa, synthetic construct
GGLGNDVIK

SEQ ID NO: 9702 - protein, 9 aa, synthetic construct
GGDGADSLH

SEQ ID NO: 9703 - protein, 9 aa, synthetic construct
GGNGEDTLS

SEQ ID NO: 9704 - protein, 9 aa, synthetic construct
GGSGDDKLE

SEQ ID NO: 9705 - protein, 9 aa, synthetic construct
GGSGDDLLG

SEQ ID NO: 9706 - protein, 9 aa, synthetic construct
GGGGSDTFI

SEQ ID NO: 9707 - protein, 9 aa, synthetic construct
GGKGNDVMM

SEQ ID NO: 9708 - protein, 9 aa, synthetic construct
GGDGADSVS

SEQ ID NO: 9709 - protein, 9 aa, synthetic construct
GGEGDDLFK

SEQ ID NO: 9710 - protein, 9 aa, synthetic construct
GGNGEDTLI

SEQ ID NO: 9711 - protein, 9 aa, synthetic construct
GGAGGDVIG

SEQ ID NO: 9712 - protein, 9 aa, synthetic construct
GGDGADSMA

SEQ ID NO: 9713 - protein, 9 aa, synthetic construct
GGTGGDELY

SEQ ID NO: 9714 - protein, 9 aa, synthetic construct
GGFGADLLT

SEQ ID NO: 9715 - protein, 9 aa, synthetic construct
GGSGDDKLF

SEQ ID NO: 9716 - protein, 9 aa, synthetic construct
GGSGDDLIS

SEQ ID NO: 9717 - protein, 9 aa, synthetic construct
GGSGDDLIR

SEQ ID NO: 9718 - protein, 9 aa, synthetic construct
GGSGDDLIK

SEQ ID NO: 9719 - protein, 9 aa, synthetic construct
GGTGGDILD

SEQ ID NO: 9720 - protein, 9 aa, synthetic construct
GGSGDDLFL

SEQ ID NO: 9721 - protein, 9 aa, synthetic construct
GGAGNDRVL

SEQ ID NO: 9722 - protein, 9 aa, synthetic construct
GGSGDDKVY

SEQ ID NO: 9723 - protein, 9 aa, synthetic construct
GGAGNDRVW

SEQ ID NO: 9724 - protein, 9 aa, synthetic construct
GGDGNDMLH

SEQ ID NO: 9725 - protein, 9 aa, synthetic construct
GGTGGDTLN

SEQ ID NO: 9726 - protein, 9 aa, synthetic construct
GGTGHDVFQ

SEQ ID NO: 9727 - protein, 9 aa, synthetic construct
GGYGNDSLY

SEQ ID NO: 9728 - protein, 9 aa, synthetic construct
GGAGNDSMH

SEQ ID NO: 9729 - protein, 9 aa, synthetic construct
GGFGADELQ

SEQ ID NO: 9730 - protein, 9 aa, synthetic construct
GGKGQDVIN

SEQ ID NO: 9731 - protein, 9 aa, synthetic construct
GGDGNDLYL

SEQ ID NO: 9732 - protein, 9 aa, synthetic construct
GGDGADRIV

SEQ ID NO: 9733 - protein, 9 aa, synthetic construct
GGSGDDDLV

SEQ ID NO: 9734 - protein, 9 aa, synthetic construct
GGDGEDRLS

SEQ ID NO: 9735 - protein, 9 aa, synthetic construct
GGNGNDSII

SEQ ID NO: 9736 - protein, 9 aa, synthetic construct
GGDGNDLVY

SEQ ID NO: 9737 - protein, 9 aa, synthetic construct
GGFGADDLR

SEQ ID NO: 9738 - protein, 9 aa, synthetic construct
GGAGGDQIN

SEQ ID NO: 9739 - protein, 9 aa, synthetic construct
GGIGNDIYV

SEQ ID NO: 9740 - protein, 9 aa, synthetic construct
GGEGADIFD

SEQ ID NO: 9741 - protein, 9 aa, synthetic construct
GGSGDDAIS

SEQ ID NO: 9742 - protein, 9 aa, synthetic construct
GGAGNDSYT

SEQ ID NO: 9743 - protein, 9 aa, synthetic construct
GGDGADRIL

SEQ ID NO: 9744 - protein, 9 aa, synthetic construct
GGSGADYLS

SEQ ID NO: 9745 - protein, 9 aa, synthetic construct
GGIGNDILY

SEQ ID NO: 9746 - protein, 9 aa, synthetic construct
GGTGHDTVS

SEQ ID NO: 9747 - protein, 9 aa, synthetic construct
GGTGHDLLQ

SEQ ID NO: 9748 - protein, 9 aa, synthetic construct
GGSGDDEIN

SEQ ID NO: 9749 - protein, 9 aa, synthetic construct
GGAGNDSMA

SEQ ID NO: 9750 - protein, 9 aa, synthetic construct
GGNGRDIVR

SEQ ID NO: 9751 - protein, 9 aa, synthetic construct
GGEGDDWLD

SEQ ID NO: 9752 - protein, 9 aa, synthetic construct
GGNGNDSIT

SEQ ID NO: 9753 - protein, 9 aa, synthetic construct
GGAGGDSLH

SEQ ID NO: 9754 - protein, 9 aa, synthetic construct
GGEGDDWLE

SEQ ID NO: 9755 - protein, 9 aa, synthetic construct
GGGGSDKLN

SEQ ID NO: 9756 - protein, 9 aa, synthetic construct
GGSGDDFLE

SEQ ID NO: 9757 - protein, 9 aa, synthetic construct
GGIGNDLLS

SEQ ID NO: 9758 - protein, 9 aa, synthetic construct
GGMGADMLL

SEQ ID NO: 9759 - protein, 9 aa, synthetic construct
GGEGNDLIK

SEQ ID NO: 9760 - protein, 9 aa, synthetic construct
GGSGDDEIY

SEQ ID NO: 9761 - protein, 9 aa, synthetic construct
GGDGHDILY

SEQ ID NO: 9762 - protein, 9 aa, synthetic construct
GGAGGDRLV

SEQ ID NO: 9763 - protein, 9 aa, synthetic construct
GGNGADVFV

SEQ ID NO: 9764 - protein, 9 aa, synthetic construct
GGMGADLMD

SEQ ID NO: 9765 - protein, 9 aa, synthetic construct
GGSGDDELS

SEQ ID NO: 9766 - protein, 9 aa, synthetic construct
GGTGHDIVY

SEQ ID NO: 9767 - protein, 9 aa, synthetic construct
GGSGDDELL

SEQ ID NO: 9768 - protein, 9 aa, synthetic construct
GGTGHDLLD

SEQ ID NO: 9769 - protein, 9 aa, synthetic construct
GGGGTDRLE

SEQ ID NO: 9770 - protein, 9 aa, synthetic construct
GGGGDDVLM

SEQ ID NO: 9771 - protein, 9 aa, synthetic construct
GGIGDDEMH

SEQ ID NO: 9772 - protein, 9 aa, synthetic construct
GGAGSDVYI

SEQ ID NO: 9773 - protein, 9 aa, synthetic construct
GGDGTDTID

SEQ ID NO: 9774 - protein, 9 aa, synthetic construct
GGAGSDVLQ

SEQ ID NO: 9775 - protein, 9 aa, synthetic construct
GGWGDDLLI

SEQ ID NO: 9776 - protein, 9 aa, synthetic construct
GGQGDDSLN

SEQ ID NO: 9777 - protein, 9 aa, synthetic construct
GGAGSDVMI

SEQ ID NO: 9778 - protein, 9 aa, synthetic construct
GGDGTDTIT

SEQ ID NO: 9779 - protein, 9 aa, synthetic construct
GGEGGDDLS

SEQ ID NO: 9780 - protein, 9 aa, synthetic construct
GGAGVDTID

SEQ ID NO: 9781 - protein, 9 aa, synthetic construct
GGMGNDSVH

SEQ ID NO: 9782 - protein, 9 aa, synthetic construct
GGQGDDRLF

SEQ ID NO: 9783 - protein, 9 aa, synthetic construct
GGEGSDLIF

SEQ ID NO: 9784 - protein, 9 aa, synthetic construct
GGDGDDVVN

SEQ ID NO: 9785 - protein, 9 aa, synthetic construct
GGQGDDQLY

SEQ ID NO: 9786 - protein, 9 aa, synthetic construct
GGAGDDGLN

SEQ ID NO: 9787 - protein, 9 aa, synthetic construct
GGDGKDTLT

SEQ ID NO: 9788 - protein, 9 aa, synthetic construct
GGPGHDTLI

SEQ ID NO: 9789 - protein, 9 aa, synthetic construct
GGAGSDWLD

SEQ ID NO: 9790 - protein, 9 aa, synthetic construct
GGDGKDTLN

SEQ ID NO: 9791 - protein, 9 aa, synthetic construct
GGDGKDTLL

SEQ ID NO: 9792 - protein, 9 aa, synthetic construct
GGDGDDAIS

SEQ ID NO: 9793 - protein, 9 aa, synthetic construct
GGQGDDTIE

SEQ ID NO: 9794 - protein, 9 aa, synthetic construct
GGQGDDTII

SEQ ID NO: 9795 - protein, 9 aa, synthetic construct
GGWGDDRID

SEQ ID NO: 9796 - protein, 9 aa, synthetic construct
GGAGDDHLT

SEQ ID NO: 9797 - protein, 9 aa, synthetic construct
GGAGDDIFE

SEQ ID NO: 9798 - protein, 9 aa, synthetic construct
GGLGNDDLN

SEQ ID NO: 9799 - protein, 9 aa, synthetic construct
GGQGDDVIL

SEQ ID NO: 9800 - protein, 9 aa, synthetic construct
GGEGSDLIE

SEQ ID NO: 9801 - protein, 9 aa, synthetic construct
GGQGDDVID

SEQ ID NO: 9802 - protein, 9 aa, synthetic construct
GGWGDDTLL

SEQ ID NO: 9803 - protein, 9 aa, synthetic construct
GGAGSDVIV

SEQ ID NO: 9804 - protein, 9 aa, synthetic construct
GGQGDDTYN

SEQ ID NO: 9805 - protein, 9 aa, synthetic construct
GGAGVDTMD

SEQ ID NO: 9806 - protein, 9 aa, synthetic construct
GGDGDDALN

SEQ ID NO: 9807 - protein, 9 aa, synthetic construct
GGQGDDTVV

SEQ ID NO: 9808 - protein, 9 aa, synthetic construct
GGAGADTAW

SEQ ID NO: 9809 - protein, 9 aa, synthetic construct
GGQGDDTVL

SEQ ID NO: 9810 - protein, 9 aa, synthetic construct
GGAGSDVLH

SEQ ID NO: 9811 - protein, 9 aa, synthetic construct
GGAGDDHVF

SEQ ID NO: 9812 - protein, 9 aa, synthetic construct
GGVGKDSLN

SEQ ID NO: 9813 - protein, 9 aa, synthetic construct
GGEGNDTVT

SEQ ID NO: 9814 - protein, 9 aa, synthetic construct
GGAGDDHLW

SEQ ID NO: 9815 - protein, 9 aa, synthetic construct
GGPGHDLLY

SEQ ID NO: 9816 - protein, 9 aa, synthetic construct
GGLGFDRLF

SEQ ID NO: 9817 - protein, 9 aa, synthetic construct
GGWGDDILD

SEQ ID NO: 9818 - protein, 9 aa, synthetic construct
GGGGGDTLA

SEQ ID NO: 9819 - protein, 9 aa, synthetic construct
GGAGDDFLE

SEQ ID NO: 9820 - protein, 9 aa, synthetic construct
GGNGNDALS

SEQ ID NO: 9821 - protein, 9 aa, synthetic construct
GGLGQDILT

SEQ ID NO: 9822 - protein, 9 aa, synthetic construct
GGLGQDILV

SEQ ID NO: 9823 - protein, 9 aa, synthetic construct
GGGGNDAFI

SEQ ID NO: 9824 - protein, 9 aa, synthetic construct
GGVGNDLFI

SEQ ID NO: 9825 - protein, 9 aa, synthetic construct
GGMGNDMLN

SEQ ID NO: 9826 - protein, 9 aa, synthetic construct
GGGGRDRLN

SEQ ID NO: 9827 - protein, 9 aa, synthetic construct
GGGGDDELD

SEQ ID NO: 9828 - protein, 9 aa, synthetic construct
GGEGDDFIY

SEQ ID NO: 9829 - protein, 9 aa, synthetic construct
GGDGKDNFL

SEQ ID NO: 9830 - protein, 9 aa, synthetic construct
GGGGMDTLY

SEQ ID NO: 9831 - protein, 9 aa, synthetic construct
GGWGADVMS

SEQ ID NO: 9832 - protein, 9 aa, synthetic construct
GGAGTDIAV

SEQ ID NO: 9833 - protein, 9 aa, synthetic construct
GGEGFDTFL

SEQ ID NO: 9834 - protein, 9 aa, synthetic construct
GGLGQDVFD

SEQ ID NO: 9835 - protein, 9 aa, synthetic construct
GGQGADTMA

SEQ ID NO: 9836 - protein, 9 aa, synthetic construct
GGEGNDVFV

SEQ ID NO: 9837 - protein, 9 aa, synthetic construct
GGWGADTMI

SEQ ID NO: 9838 - protein, 9 aa, synthetic construct
GGLGNDAIN

SEQ ID NO: 9839 - protein, 9 aa, synthetic construct
GGVGNDIYI

SEQ ID NO: 9840 - protein, 9 aa, synthetic construct
GGWGDDFLS

SEQ ID NO: 9841 - protein, 9 aa, synthetic construct
GGQGDDLLR

SEQ ID NO: 9842 - protein, 9 aa, synthetic construct
GGVGNDILS

SEQ ID NO: 9843 - protein, 9 aa, synthetic construct
GGQGDDLLL

SEQ ID NO: 9844 - protein, 9 aa, synthetic construct
GGDGTDTVS

SEQ ID NO: 9845 - protein, 9 aa, synthetic construct
GGDGTDTVV

SEQ ID NO: 9846 - protein, 9 aa, synthetic construct
GGVGNDELS

SEQ ID NO: 9847 - protein, 9 aa, synthetic construct
GGDGTDVIY

SEQ ID NO: 9848 - protein, 9 aa, synthetic construct
GGEGSDIFV

SEQ ID NO: 9849 - protein, 9 aa, synthetic construct
GGGGDDALS

SEQ ID NO: 9850 - protein, 9 aa, synthetic construct
GGWGDDILC

SEQ ID NO: 9851 - protein, 9 aa, synthetic construct
GGGGNDAIY

SEQ ID NO: 9852 - protein, 9 aa, synthetic construct
GGQGDDILR

SEQ ID NO: 9853 - protein, 9 aa, synthetic construct
GGVGNDFLN

SEQ ID NO: 9854 - protein, 9 aa, synthetic construct
GGQGDDILD

SEQ ID NO: 9855 - protein, 9 aa, synthetic construct
GGNGNDAFV

SEQ ID NO: 9856 - protein, 9 aa, synthetic construct
GGDGCDYID

SEQ ID NO: 9857 - protein, 9 aa, synthetic construct
GGGGNDAIS

SEQ ID NO: 9858 - protein, 9 aa, synthetic construct
GGGGRDRLA

SEQ ID NO: 9859 - protein, 9 aa, synthetic construct
GGAGDDFLV

SEQ ID NO: 9860 - protein, 9 aa, synthetic construct
GGGGRDRLE

SEQ ID NO: 9861 - protein, 9 aa, synthetic construct
GGVGNDILL

SEQ ID NO: 9862 - protein, 9 aa, synthetic construct
GGAGDDIFF

SEQ ID NO: 9863 - protein, 9 aa, synthetic construct
GGDGDDALV

SEQ ID NO: 9864 - protein, 9 aa, synthetic construct
GGEGNDVIE

SEQ ID NO: 9865 - protein, 9 aa, synthetic construct
GGQGIDWVS

SEQ ID NO: 9866 - protein, 9 aa, synthetic construct
GGLGDDVLE

SEQ ID NO: 9867 - protein, 9 aa, synthetic construct
GGVGDDTYY

SEQ ID NO: 9868 - protein, 9 aa, synthetic construct
GGAGDDLIG

SEQ ID NO: 9869 - protein, 9 aa, synthetic construct
GGGGADVIR

SEQ ID NO: 9870 - protein, 9 aa, synthetic construct
GGLGDDVLK

SEQ ID NO: 9871 - protein, 9 aa, synthetic construct
GGVGDDVIS

SEQ ID NO: 9872 - protein, 9 aa, synthetic construct
GGGGVDTLT

SEQ ID NO: 9873 - protein, 9 aa, synthetic construct
GGGGDDRID

SEQ ID NO: 9874 - protein, 9 aa, synthetic construct
GGVGDDVLL

SEQ ID NO: 9875 - protein, 9 aa, synthetic construct
GGAGDDLFR

SEQ ID NO: 9876 - protein, 9 aa, synthetic construct
GGLGNDDLR

SEQ ID NO: 9877 - protein, 9 aa, synthetic construct
GGVGDDVYI

SEQ ID NO: 9878 - protein, 9 aa, synthetic construct
GGAGDDLFI

SEQ ID NO: 9879 - protein, 9 aa, synthetic construct
GGQGIDTLD

SEQ ID NO: 9880 - protein, 9 aa, synthetic construct
GGAGSDSLE

SEQ ID NO: 9881 - protein, 9 aa, synthetic construct
GGDGDDDID

SEQ ID NO: 9882 - protein, 9 aa, synthetic construct
GGVGDDYLN

SEQ ID NO: 9883 - protein, 9 aa, synthetic construct
GGWGEDLLY

SEQ ID NO: 9884 - protein, 9 aa, synthetic construct
GGLGDDVMI

SEQ ID NO: 9885 - protein, 9 aa, synthetic construct
GGGGNDELY

SEQ ID NO: 9886 - protein, 9 aa, synthetic construct
GGMGNDVLY

SEQ ID NO: 9887 - protein, 9 aa, synthetic construct
GGAGDDLIH

SEQ ID NO: 9888 - protein, 9 aa, synthetic construct
GGAGADSIG

SEQ ID NO: 9889 - protein, 9 aa, synthetic construct
GGAGSDRMS

SEQ ID NO: 9890 - protein, 9 aa, synthetic construct
GGQGNDELW

SEQ ID NO: 9891 - protein, 9 aa, synthetic construct
GGQGNDEID

SEQ ID NO: 9892 - protein, 9 aa, synthetic construct
GGAGSDQIY

SEQ ID NO: 9893 - protein, 9 aa, synthetic construct
GGGGADVFI

SEQ ID NO: 9894 - protein, 9 aa, synthetic construct
GGAGSDQLI

SEQ ID NO: 9895 - protein, 9 aa, synthetic construct
GGVGDDRLN

SEQ ID NO: 9896 - protein, 9 aa, synthetic construct
GGLGNDFLS

SEQ ID NO: 9897 - protein, 9 aa, synthetic construct
GGQGNDALF

SEQ ID NO: 9898 - protein, 9 aa, synthetic construct
GGLGNDFLQ

SEQ ID NO: 9899 - protein, 9 aa, synthetic construct
GGVGDDSLT

SEQ ID NO: 9900 - protein, 9 aa, synthetic construct
GGDGGDTIS

SEQ ID NO: 9901 - protein, 9 aa, synthetic construct
GGNGKDTLY

SEQ ID NO: 9902 - protein, 9 aa, synthetic construct
GGQGLDRLF

SEQ ID NO: 9903 - protein, 9 aa, synthetic construct
GGHGNDTLI

SEQ ID NO: 9904 - protein, 9 aa, synthetic construct
GGVGDDTIN

SEQ ID NO: 9905 - protein, 9 aa, synthetic construct
GGAGSDRLN

SEQ ID NO: 9906 - protein, 9 aa, synthetic construct
GGGGVDTLN

SEQ ID NO: 9907 - protein, 9 aa, synthetic construct
GGDGADVLV

SEQ ID NO: 9908 - protein, 9 aa, synthetic construct
GGAGDDLIK

SEQ ID NO: 9909 - protein, 9 aa, synthetic construct
GGEGSDNIF

SEQ ID NO: 9910 - protein, 9 aa, synthetic construct
GGHGNDRIF

SEQ ID NO: 9911 - protein, 9 aa, synthetic construct
GGVGEDLLI

SEQ ID NO: 9912 - protein, 9 aa, synthetic construct
GGEGSDLLR

SEQ ID NO: 9913 - protein, 9 aa, synthetic construct
GGMGNDTLV

SEQ ID NO: 9914 - protein, 9 aa, synthetic construct
GGDGEDVLY

SEQ ID NO: 9915 - protein, 9 aa, synthetic construct
GGEGDDELI

SEQ ID NO: 9916 - protein, 9 aa, synthetic construct
GGMGNDTLS

SEQ ID NO: 9917 - protein, 9 aa, synthetic construct
GGGGNDDLY

SEQ ID NO: 9918 - protein, 9 aa, synthetic construct
GGLGEDELY

SEQ ID NO: 9919 - protein, 9 aa, synthetic construct
GGAGDDIVI

SEQ ID NO: 9920 - protein, 9 aa, synthetic construct
GGAGSDTVT

SEQ ID NO: 9921 - protein, 9 aa, synthetic construct
GGAGSDTYI

SEQ ID NO: 9922 - protein, 9 aa, synthetic construct
GGGGDDQLT

SEQ ID NO: 9923 - protein, 9 aa, synthetic construct
GGDGGDTLT

SEQ ID NO: 9924 - protein, 9 aa, synthetic construct
GGQGDDYLS

SEQ ID NO: 9925 - protein, 9 aa, synthetic construct
GGQGDDYID

SEQ ID NO: 9926 - protein, 9 aa, synthetic construct
GGHGNDFLN

SEQ ID NO: 9927 - protein, 9 aa, synthetic construct
GGAGSDVFA

SEQ ID NO: 9928 - protein, 9 aa, synthetic construct
GGAGDDIIQ

SEQ ID NO: 9929 - protein, 9 aa, synthetic construct
GGAGDDIIL

SEQ ID NO: 9930 - protein, 9 aa, synthetic construct
GGAGVDTVN

SEQ ID NO: 9931 - protein, 9 aa, synthetic construct
GGAGVDTVL

SEQ ID NO: 9932 - protein, 9 aa, synthetic construct
GGHGNDILD

SEQ ID NO: 9933 - protein, 9 aa, synthetic construct
GGAGVDVLL

SEQ ID NO: 9934 - protein, 9 aa, synthetic construct
GGGGADVLY

SEQ ID NO: 9935 - protein, 9 aa, synthetic construct
GGQGGDALF

SEQ ID NO: 9936 - protein, 9 aa, synthetic construct
GGDGEDELY

SEQ ID NO: 9937 - protein, 9 aa, synthetic construct
GGAGSDSYI

SEQ ID NO: 9938 - protein, 9 aa, synthetic construct
GGVGEDQYL

SEQ ID NO: 9939 - protein, 9 aa, synthetic construct
GGMGNDTYY

SEQ ID NO: 9940 - protein, 9 aa, synthetic construct
GGAGSDTAI

SEQ ID NO: 9941 - protein, 9 aa, synthetic construct
GGGGADVMR

SEQ ID NO: 9942 - protein, 9 aa, synthetic construct
GGGGADVMT

SEQ ID NO: 9943 - protein, 9 aa, synthetic construct
GGVGEDTFI

SEQ ID NO: 9944 - protein, 9 aa, synthetic construct
GGVGEDTIH

SEQ ID NO: 9945 - protein, 9 aa, synthetic construct
GGQGGDWLY

SEQ ID NO: 9946 - protein, 9 aa, synthetic construct
GGDGEDVLT

SEQ ID NO: 9947 - protein, 9 aa, synthetic construct
GGEGDDEIY

SEQ ID NO: 9948 - protein, 9 aa, synthetic construct
GGAGSDTII

SEQ ID NO: 9949 - protein, 9 aa, synthetic construct
GGVGFDLLQ

SEQ ID NO: 9950 - protein, 9 aa, synthetic construct
GGAGSDTIQ

SEQ ID NO: 9951 - protein, 9 aa, synthetic construct
GGLGNDELY

SEQ ID NO: 9952 - protein, 9 aa, synthetic construct
GGNGLDELH

SEQ ID NO: 9953 - protein, 9 aa, synthetic construct
GGEGDDSLN

SEQ ID NO: 9954 - protein, 9 aa, synthetic construct
GGDGVDTVD

SEQ ID NO: 9955 - protein, 9 aa, synthetic construct
GGQGADTIS

SEQ ID NO: 9956 - protein, 9 aa, synthetic construct
GGQGADTIN

SEQ ID NO: 9957 - protein, 9 aa, synthetic construct
GGGGADLIY

SEQ ID NO: 9958 - protein, 9 aa, synthetic construct
GGHGADTIN

SEQ ID NO: 9959 - protein, 9 aa, synthetic construct
GGAGADYLV

SEQ ID NO: 9960 - protein, 9 aa, synthetic construct
GGAGADVFN

SEQ ID NO: 9961 - protein, 9 aa, synthetic construct
GGAGADYLN

SEQ ID NO: 9962 - protein, 9 aa, synthetic construct
GGEGEDVLG

SEQ ID NO: 9963 - protein, 9 aa, synthetic construct
GGEGEDVLF

SEQ ID NO: 9964 - protein, 9 aa, synthetic construct
GGAGADYLE

SEQ ID NO: 9965 - protein, 9 aa, synthetic construct
GGEGDDIFL

SEQ ID NO: 9966 - protein, 9 aa, synthetic construct
GGGGKDTID

SEQ ID NO: 9967 - protein, 9 aa, synthetic construct
GGGGKDVLT

SEQ ID NO: 9968 - protein, 9 aa, synthetic construct
GGNGNDKLS

SEQ ID NO: 9969 - protein, 9 aa, synthetic construct
GGAGDDAIF

SEQ ID NO: 9970 - protein, 9 aa, synthetic construct
GGGGDDMLS

SEQ ID NO: 9971 - protein, 9 aa, synthetic construct
GGGGDDLIF

SEQ ID NO: 9972 - protein, 9 aa, synthetic construct
GGPGNDELW

SEQ ID NO: 9973 - protein, 9 aa, synthetic construct
GGEGRDVIH

SEQ ID NO: 9974 - protein, 9 aa, synthetic construct
GGGGRDVLE

SEQ ID NO: 9975 - protein, 9 aa, synthetic construct
GGGGDDMLD

SEQ ID NO: 9976 - protein, 9 aa, synthetic construct
GGPGNDTYS

SEQ ID NO: 9977 - protein, 9 aa, synthetic construct
GGGGDDLIR

SEQ ID NO: 9978 - protein, 9 aa, synthetic construct
GGPGNDTVT

SEQ ID NO: 9979 - protein, 9 aa, synthetic construct
GGLGKDLLV

SEQ ID NO: 9980 - protein, 9 aa, synthetic construct
GGDGVDLLD

SEQ ID NO: 9981 - protein, 9 aa, synthetic construct
GGEGDDLIS

SEQ ID NO: 9982 - protein, 9 aa, synthetic construct
GGLGLDTLV

SEQ ID NO: 9983 - protein, 9 aa, synthetic construct
GGEGRDTLD

SEQ ID NO: 9984 - protein, 9 aa, synthetic construct
GGEGDDSLI

SEQ ID NO: 9985 - protein, 9 aa, synthetic construct
GGGGDDILK

SEQ ID NO: 9986 - protein, 9 aa, synthetic construct
GGGGKDTFL

SEQ ID NO: 9987 - protein, 9 aa, synthetic construct
GGVGRDTIA

SEQ ID NO: 9988 - protein, 9 aa, synthetic construct
GGLGVDTLA

SEQ ID NO: 9989 - protein, 9 aa, synthetic construct
GGDGDDYIR

SEQ ID NO: 9990 - protein, 9 aa, synthetic construct
GGAGTDYLD

SEQ ID NO: 9991 - protein, 9 aa, synthetic construct
GGAGTDYLI

SEQ ID NO: 9992 - protein, 9 aa, synthetic construct
GGAGADVAV

SEQ ID NO: 9993 - protein, 9 aa, synthetic construct
GGGGRDVLL

SEQ ID NO: 9994 - protein, 9 aa, synthetic construct
GGAGADYMT

SEQ ID NO: 9995 - protein, 9 aa, synthetic construct
GGPGQDTLV

SEQ ID NO: 9996 - protein, 9 aa, synthetic construct
GGEGEDYIN

SEQ ID NO: 9997 - protein, 9 aa, synthetic construct
GGEGDDLIT

SEQ ID NO: 9998 - protein, 9 aa, synthetic construct
GGPGQDRLW

SEQ ID NO: 9999 - protein, 9 aa, synthetic construct
GGLGKDALT

SEQ ID NO: 10000 - protein, 9 aa, synthetic construct
GGAGADVFH

SEQ ID NO: 10001 - protein, 9 aa, synthetic construct
GGPGQDMLM

SEQ ID NO: 10002 - protein, 9 aa, synthetic construct
GGAGADWMA

SEQ ID NO: 10003 - protein, 9 aa, synthetic construct
GGEGNDVVS

SEQ ID NO: 10004 - protein, 9 aa, synthetic construct
GGGGDDLIY

SEQ ID NO: 10005 - protein, 9 aa, synthetic construct
GGEGRDTLV

SEQ ID NO: 10006 - protein, 9 aa, synthetic construct
GGGGRDVFY

SEQ ID NO: 10007 - protein, 9 aa, synthetic construct
GGLGKDVLN

SEQ ID NO: 10008 - protein, 9 aa, synthetic construct
GGPGNDQLF

SEQ ID NO: 10009 - protein, 9 aa, synthetic construct
GGPGNDILV

SEQ ID NO: 10010 - protein, 9 aa, synthetic construct
GGLGKDVLV

SEQ ID NO: 10011 - protein, 9 aa, synthetic construct
GGVGTDILS

SEQ ID NO: 10012 - protein, 9 aa, synthetic construct
GGLGKDWLY

SEQ ID NO: 10013 - protein, 9 aa, synthetic construct
GGAGADVML

SEQ ID NO: 10014 - protein, 9 aa, synthetic construct
GGGGEDTLN

SEQ ID NO: 10015 - protein, 9 aa, synthetic construct
GGAGADVMK

SEQ ID NO: 10016 - protein, 9 aa, synthetic construct
GGAGVDLVA

SEQ ID NO: 10017 - protein, 9 aa, synthetic construct
GGPGNDIMT

SEQ ID NO: 10018 - protein, 9 aa, synthetic construct
GGGGDDLVE

SEQ ID NO: 10019 - protein, 9 aa, synthetic construct
GGPGNDLLS

SEQ ID NO: 10020 - protein, 9 aa, synthetic construct
GGAGVDMAD

SEQ ID NO: 10021 - protein, 9 aa, synthetic construct
GGEGDDIIY

SEQ ID NO: 10022 - protein, 9 aa, synthetic construct
GGAGADVLW

SEQ ID NO: 10023 - protein, 9 aa, synthetic construct
GGEGDDIIS

SEQ ID NO: 10024 - protein, 9 aa, synthetic construct
GGPGNDLIF

SEQ ID NO: 10025 - protein, 9 aa, synthetic construct
GGPGNDRII

SEQ ID NO: 10026 - protein, 9 aa, synthetic construct
GGVGTDTLN

SEQ ID NO: 10027 - protein, 9 aa, synthetic construct
GGAGADWLS

SEQ ID NO: 10028 - protein, 9 aa, synthetic construct
GGVGSDVFV

SEQ ID NO: 10029 - protein, 9 aa, synthetic construct
GGAGADWLR

SEQ ID NO: 10030 - protein, 9 aa, synthetic construct
GGGGKDTIR

SEQ ID NO: 10031 - protein, 9 aa, synthetic construct
GGVGSDRLY

SEQ ID NO: 10032 - protein, 9 aa, synthetic construct
GGGGKDTIS

SEQ ID NO: 10033 - protein, 9 aa, synthetic construct
GGPGNDTLK

SEQ ID NO: 10034 - protein, 9 aa, synthetic construct
GGLGVDTLV

SEQ ID NO: 10035 - protein, 9 aa, synthetic construct
GGDGDDYLL

SEQ ID NO: 10036 - protein, 9 aa, synthetic construct
GGPGNDTIR

SEQ ID NO: 10037 - protein, 9 aa, synthetic construct
GGEGDDILA

SEQ ID NO: 10038 - protein, 9 aa, synthetic construct
GGPGNDTIH

SEQ ID NO: 10039 - protein, 9 aa, synthetic construct
GGGGDDLLE

SEQ ID NO: 10040 - protein, 9 aa, synthetic construct
GGPGNDSLV

SEQ ID NO: 10041 - protein, 9 aa, synthetic construct
GGPGNDHLY

SEQ ID NO: 10042 - protein, 9 aa, synthetic construct
GGVGSDTLD

SEQ ID NO: 10043 - protein, 9 aa, synthetic construct
GGPGNDSLD

SEQ ID NO: 10044 - protein, 9 aa, synthetic construct
GGAGADVLH

SEQ ID NO: 10045 - protein, 9 aa, synthetic construct
GGLGKDTLY

SEQ ID NO: 10046 - protein, 9 aa, synthetic construct
GGEGDDIIE

SEQ ID NO: 10047 - protein, 9 aa, synthetic construct
GGAGADWFA

SEQ ID NO: 10048 - protein, 9 aa, synthetic construct
GGAGTDVLY

SEQ ID NO: 10049 - protein, 9 aa, synthetic construct
GGHGDDHLN

SEQ ID NO: 10050 - protein, 9 aa, synthetic construct
GGLGGDTIS

SEQ ID NO: 10051 - protein, 9 aa, synthetic construct
GGGGYDIYV

SEQ ID NO: 10052 - protein, 9 aa, synthetic construct
GGVGNDRLT

SEQ ID NO: 10053 - protein, 9 aa, synthetic construct
GGLGQDILW

SEQ ID NO: 10054 - protein, 9 aa, synthetic construct
GGAGDDEIW

SEQ ID NO: 10055 - protein, 9 aa, synthetic construct
GGDGVDTFV

SEQ ID NO: 10056 - protein, 9 aa, synthetic construct
GGQGADLMV

SEQ ID NO: 10057 - protein, 9 aa, synthetic construct
GGNGNDELH

SEQ ID NO: 10058 - protein, 9 aa, synthetic construct
GGAGVDSLF

SEQ ID NO: 10059 - protein, 9 aa, synthetic construct
GGPGKDLLE

SEQ ID NO: 10060 - protein, 9 aa, synthetic construct
GGAGTDLVE

SEQ ID NO: 10061 - protein, 9 aa, synthetic construct
GGEGDDILQ

SEQ ID NO: 10062 - protein, 9 aa, synthetic construct
GGDGVDILV

SEQ ID NO: 10063 - protein, 9 aa, synthetic construct
GGDGADYLR

SEQ ID NO: 10064 - protein, 9 aa, synthetic construct
GGAGDDEII

SEQ ID NO: 10065 - protein, 9 aa, synthetic construct
GGGGDDFMI

SEQ ID NO: 10066 - protein, 9 aa, synthetic construct
GGQGADIFV

SEQ ID NO: 10067 - protein, 9 aa, synthetic construct
GGAGVDSID

SEQ ID NO: 10068 - protein, 9 aa, synthetic construct
GGDGFDAIG

SEQ ID NO: 10069 - protein, 9 aa, synthetic construct
GGGGLDVLD

SEQ ID NO: 10070 - protein, 9 aa, synthetic construct
GGAGTDNYY

SEQ ID NO: 10071 - protein, 9 aa, synthetic construct
GGLGHDHLR

SEQ ID NO: 10072 - protein, 9 aa, synthetic construct
GGVGNDRLN

SEQ ID NO: 10073 - protein, 9 aa, synthetic construct
GGVGNDRLE

SEQ ID NO: 10074 - protein, 9 aa, synthetic construct
GGQGADQLN

SEQ ID NO: 10075 - protein, 9 aa, synthetic construct
GGMGNDKYI

SEQ ID NO: 10076 - protein, 9 aa, synthetic construct
GGGGKDRLT

SEQ ID NO: 10077 - protein, 9 aa, synthetic construct
GGAGTDILS

SEQ ID NO: 10078 - protein, 9 aa, synthetic construct
GGAGTDILV

SEQ ID NO: 10079 - protein, 9 aa, synthetic construct
GGNGNDLIE

SEQ ID NO: 10080 - protein, 9 aa, synthetic construct
GGMGNDLLN

SEQ ID NO: 10081 - protein, 9 aa, synthetic construct
GGQGADSMT

SEQ ID NO: 10082 - protein, 9 aa, synthetic construct
GGEGNDVIN

SEQ ID NO: 10083 - protein, 9 aa, synthetic construct
GGQGADSMA

SEQ ID NO: 10084 - protein, 9 aa, synthetic construct
GGWGADRFY

SEQ ID NO: 10085 - protein, 9 aa, synthetic construct
GGLGGDTLS

SEQ ID NO: 10086 - protein, 9 aa, synthetic construct
GGMGNDLLI

SEQ ID NO: 10087 - protein, 9 aa, synthetic construct
GGAGADTVE

SEQ ID NO: 10088 - protein, 9 aa, synthetic construct
GGEGDDVLQ

SEQ ID NO: 10089 - protein, 9 aa, synthetic construct
GGAGADTVF

SEQ ID NO: 10090 - protein, 9 aa, synthetic construct
GGVGNDQLY

SEQ ID NO: 10091 - protein, 9 aa, synthetic construct
GGGGDDFIR

SEQ ID NO: 10092 - protein, 9 aa, synthetic construct
GGAGTDLAS

SEQ ID NO: 10093 - protein, 9 aa, synthetic construct
GGGGDDFLA

SEQ ID NO: 10094 - protein, 9 aa, synthetic construct
GGDGKDKLW

SEQ ID NO: 10095 - protein, 9 aa, synthetic construct
GGAGDDEIA

SEQ ID NO: 10096 - protein, 9 aa, synthetic construct
GGGGLDTMI

SEQ ID NO: 10097 - protein, 9 aa, synthetic construct
GGAGADTVR

SEQ ID NO: 10098 - protein, 9 aa, synthetic construct
GGVGNDWAE

SEQ ID NO: 10099 - protein, 9 aa, synthetic construct
GGVGNDWLV

SEQ ID NO: 10100 - protein, 9 aa, synthetic construct
GGDGIDTVN

SEQ ID NO: 10101 - protein, 9 aa, synthetic construct
GGPGKDYLS

SEQ ID NO: 10102 - protein, 9 aa, synthetic construct
GGVGNDYLN

SEQ ID NO: 10103 - protein, 9 aa, synthetic construct
GGHGDDLLI

SEQ ID NO: 10104 - protein, 9 aa, synthetic construct
GGAGDDAVD

SEQ ID NO: 10105 - protein, 9 aa, synthetic construct
GGEGDDLIY

SEQ ID NO: 10106 - protein, 9 aa, synthetic construct
GGPGRDVLR

SEQ ID NO: 10107 - protein, 9 aa, synthetic construct
GGGGGDTLY

SEQ ID NO: 10108 - protein, 9 aa, synthetic construct
GGDGIDTLN

SEQ ID NO: 10109 - protein, 9 aa, synthetic construct
GGAGDDALW

SEQ ID NO: 10110 - protein, 9 aa, synthetic construct
GGLGIDRLI

SEQ ID NO: 10111 - protein, 9 aa, synthetic construct
GGAGTDTYD

SEQ ID NO: 10112 - protein, 9 aa, synthetic construct
GGPGRDTLL

SEQ ID NO: 10113 - protein, 9 aa, synthetic construct
GGPGRDSLH

SEQ ID NO: 10114 - protein, 9 aa, synthetic construct
GGGGKDTFK

SEQ ID NO: 10115 - protein, 9 aa, synthetic construct
GGHGDDIIS

SEQ ID NO: 10116 - protein, 9 aa, synthetic construct
GGNGNDHLE

SEQ ID NO: 10117 - protein, 9 aa, synthetic construct
GGGGHDMLS

SEQ ID NO: 10118 - protein, 9 aa, synthetic construct
GGAGDDDIA

SEQ ID NO: 10119 - protein, 9 aa, synthetic construct
GGPGSDTAS

SEQ ID NO: 10120 - protein, 9 aa, synthetic construct
GGQGADALI

SEQ ID NO: 10121 - protein, 9 aa, synthetic construct
GGPGSDTFV

SEQ ID NO: 10122 - protein, 9 aa, synthetic construct
GGHGDDSLF

SEQ ID NO: 10123 - protein, 9 aa, synthetic construct
GGVGNDTMN

SEQ ID NO: 10124 - protein, 9 aa, synthetic construct
GGAGTDRLH

SEQ ID NO: 10125 - protein, 9 aa, synthetic construct
GGAGTDRLN

SEQ ID NO: 10126 - protein, 9 aa, synthetic construct
GGVGNDTVR

SEQ ID NO: 10127 - protein, 9 aa, synthetic construct
GGDGVDTAS

SEQ ID NO: 10128 - protein, 9 aa, synthetic construct
GGAGADTVY

SEQ ID NO: 10129 - protein, 9 aa, synthetic construct
GGGGLDTIS

SEQ ID NO: 10130 - protein, 9 aa, synthetic construct
GGMGNDILD

SEQ ID NO: 10131 - protein, 9 aa, synthetic construct
GGAGDDDLI

SEQ ID NO: 10132 - protein, 9 aa, synthetic construct
GGGGRDVLV

SEQ ID NO: 10133 - protein, 9 aa, synthetic construct
GGDGADYIS

SEQ ID NO: 10134 - protein, 9 aa, synthetic construct
GGVGNDVLF

SEQ ID NO: 10135 - protein, 9 aa, synthetic construct
GGLGHDVLD

SEQ ID NO: 10136 - protein, 9 aa, synthetic construct
GGMGGDTLI

SEQ ID NO: 10137 - protein, 9 aa, synthetic construct
GGHGDDQLH

SEQ ID NO: 10138 - protein, 9 aa, synthetic construct
GGVGNDVLR

SEQ ID NO: 10139 - protein, 9 aa, synthetic construct
GGPGSDTLV

SEQ ID NO: 10140 - protein, 9 aa, synthetic construct
GGPGSDTLD

SEQ ID NO: 10141 - protein, 9 aa, synthetic construct
GGDGLDRLY

SEQ ID NO: 10142 - protein, 9 aa, synthetic construct
GGPGDDYLD

SEQ ID NO: 10143 - protein, 9 aa, synthetic construct
GGAGADSIE

SEQ ID NO: 10144 - protein, 9 aa, synthetic construct
GGRGADTMI

SEQ ID NO: 10145 - protein, 9 aa, synthetic construct
GGTGSDTYI

SEQ ID NO: 10146 - protein, 9 aa, synthetic construct
GGRGADVLT

SEQ ID NO: 10147 - protein, 9 aa, synthetic construct
GGYGADTFT

SEQ ID NO: 10148 - protein, 9 aa, synthetic construct
GGEGSDTYY

SEQ ID NO: 10149 - protein, 9 aa, synthetic construct
GGLGNDMLS

SEQ ID NO: 10150 - protein, 9 aa, synthetic construct
GGTGSDVLD

SEQ ID NO: 10151 - protein, 9 aa, synthetic construct
GGCGNDSIS

SEQ ID NO: 10152 - protein, 9 aa, synthetic construct
GGTGSDVLT

SEQ ID NO: 10153 - protein, 9 aa, synthetic construct
GGAGDDVFF

SEQ ID NO: 10154 - protein, 9 aa, synthetic construct
GGPGADRLF

SEQ ID NO: 10155 - protein, 9 aa, synthetic construct
GGGGKDKLD

SEQ ID NO: 10156 - protein, 9 aa, synthetic construct
GGAGDDVAY

SEQ ID NO: 10157 - protein, 9 aa, synthetic construct
GGPGADRLY

SEQ ID NO: 10158 - protein, 9 aa, synthetic construct
GGLGNDLYI

SEQ ID NO: 10159 - protein, 9 aa, synthetic construct
GGLGNDLYF

SEQ ID NO: 10160 - protein, 9 aa, synthetic construct
GGAGDDTYR

SEQ ID NO: 10161 - protein, 9 aa, synthetic construct
GGAGRDTIL

SEQ ID NO: 10162 - protein, 9 aa, synthetic construct
GGGGHDRLY

SEQ ID NO: 10163 - protein, 9 aa, synthetic construct
GGIGADRLI

SEQ ID NO: 10164 - protein, 9 aa, synthetic construct
GGAGDDTYH

SEQ ID NO: 10165 - protein, 9 aa, synthetic construct
GGLGDDFLT

SEQ ID NO: 10166 - protein, 9 aa, synthetic construct
GGLGNDMLY

SEQ ID NO: 10167 - protein, 9 aa, synthetic construct
GGAGRDSMY

SEQ ID NO: 10168 - protein, 9 aa, synthetic construct
GGDGNDAIS

SEQ ID NO: 10169 - protein, 9 aa, synthetic construct
GGDGGDRLL

SEQ ID NO: 10170 - protein, 9 aa, synthetic construct
GGAGRDRVL

SEQ ID NO: 10171 - protein, 9 aa, synthetic construct
GGLGNDNLI

SEQ ID NO: 10172 - protein, 9 aa, synthetic construct
GGTGSDTAE

SEQ ID NO: 10173 - protein, 9 aa, synthetic construct
GGEGGDTLF

SEQ ID NO: 10174 - protein, 9 aa, synthetic construct
GGYGADTLS

SEQ ID NO: 10175 - protein, 9 aa, synthetic construct
GGPGADLLI

SEQ ID NO: 10176 - protein, 9 aa, synthetic construct
GGTGSDTIA

SEQ ID NO: 10177 - protein, 9 aa, synthetic construct
GGTGSDTIE

SEQ ID NO: 10178 - protein, 9 aa, synthetic construct
GGDGNDALA

SEQ ID NO: 10179 - protein, 9 aa, synthetic construct
GGLGDDFID

SEQ ID NO: 10180 - protein, 9 aa, synthetic construct
GGTGSDTIL

SEQ ID NO: 10181 - protein, 9 aa, synthetic construct
GGRGDDALS

SEQ ID NO: 10182 - protein, 9 aa, synthetic construct
GGNGNDQLR

SEQ ID NO: 10183 - protein, 9 aa, synthetic construct
GGDGHDRIF

SEQ ID NO: 10184 - protein, 9 aa, synthetic construct
GGEGNDYME

SEQ ID NO: 10185 - protein, 9 aa, synthetic construct
GGTGSDTLK

SEQ ID NO: 10186 - protein, 9 aa, synthetic construct
GGTGSDTLQ

SEQ ID NO: 10187 - protein, 9 aa, synthetic construct
GGTGSDTMI

SEQ ID NO: 10188 - protein, 9 aa, synthetic construct
GGRGADSLL

SEQ ID NO: 10189 - protein, 9 aa, synthetic construct
GGLGNDLVY

SEQ ID NO: 10190 - protein, 9 aa, synthetic construct
GGIGADRLE

SEQ ID NO: 10191 - protein, 9 aa, synthetic construct
GGRGADKLH

SEQ ID NO: 10192 - protein, 9 aa, synthetic construct
GGRGADILG

SEQ ID NO: 10193 - protein, 9 aa, synthetic construct
GGAGDDTIG

SEQ ID NO: 10194 - protein, 9 aa, synthetic construct
GGRGADHLE

SEQ ID NO: 10195 - protein, 9 aa, synthetic construct
GGEGADKLD

SEQ ID NO: 10196 - protein, 9 aa, synthetic construct
GGGGDDTIV

SEQ ID NO: 10197 - protein, 9 aa, synthetic construct
GGNGIDTAV

SEQ ID NO: 10198 - protein, 9 aa, synthetic construct
GGAGADNMT

SEQ ID NO: 10199 - protein, 9 aa, synthetic construct
GGRGADAMY

SEQ ID NO: 10200 - protein, 9 aa, synthetic construct
GGGGFDTAS

SEQ ID NO: 10201 - protein, 9 aa, synthetic construct
GGAGRDVLE

SEQ ID NO: 10202 - protein, 9 aa, synthetic construct
GGQGYDVLI

SEQ ID NO: 10203 - protein, 9 aa, synthetic construct
GGDGWDTLF

SEQ ID NO: 10204 - protein, 9 aa, synthetic construct
GGDGSDVFK

SEQ ID NO: 10205 - protein, 9 aa, synthetic construct
GGAGDDTFD

SEQ ID NO: 10206 - protein, 9 aa, synthetic construct
GGMGDDTLS

SEQ ID NO: 10207 - protein, 9 aa, synthetic construct
GGEGSDTVS

SEQ ID NO: 10208 - protein, 9 aa, synthetic construct
GGLGNDLIR

SEQ ID NO: 10209 - protein, 9 aa, synthetic construct
GGAGDDTAV

SEQ ID NO: 10210 - protein, 9 aa, synthetic construct
GGAGDDTAT

SEQ ID NO: 10211 - protein, 9 aa, synthetic construct
GGTGTDSLF

SEQ ID NO: 10212 - protein, 9 aa, synthetic construct
GGEGADRLH

SEQ ID NO: 10213 - protein, 9 aa, synthetic construct
GGRGADSLF

SEQ ID NO: 10214 - protein, 9 aa, synthetic construct
GGLGDDILG

SEQ ID NO: 10215 - protein, 9 aa, synthetic construct
GGRGADSLD

SEQ ID NO: 10216 - protein, 9 aa, synthetic construct
GGYGADQLF

SEQ ID NO: 10217 - protein, 9 aa, synthetic construct
GGAGADMLF

SEQ ID NO: 10218 - protein, 9 aa, synthetic construct
GGAGADMLN

SEQ ID NO: 10219 - protein, 9 aa, synthetic construct
GGRGADRMI

SEQ ID NO: 10220 - protein, 9 aa, synthetic construct
GGPGADTLR

SEQ ID NO: 10221 - protein, 9 aa, synthetic construct
GGEGDDAVD

SEQ ID NO: 10222 - protein, 9 aa, synthetic construct
GGEGADRLN

SEQ ID NO: 10223 - protein, 9 aa, synthetic construct
GGPGADTLS

SEQ ID NO: 10224 - protein, 9 aa, synthetic construct
GGAGDDTMR

SEQ ID NO: 10225 - protein, 9 aa, synthetic construct
GGAGDDTML

SEQ ID NO: 10226 - protein, 9 aa, synthetic construct
GGDGEDLIH

SEQ ID NO: 10227 - protein, 9 aa, synthetic construct
GGRGADNYY

SEQ ID NO: 10228 - protein, 9 aa, synthetic construct
GGNGIDRLY

SEQ ID NO: 10229 - protein, 9 aa, synthetic construct
GGLGDDIID

SEQ ID NO: 10230 - protein, 9 aa, synthetic construct
GGLGDDIIF

SEQ ID NO: 10231 - protein, 9 aa, synthetic construct
GGYGADEIS

SEQ ID NO: 10232 - protein, 9 aa, synthetic construct
GGTGTDQLS

SEQ ID NO: 10233 - protein, 9 aa, synthetic construct
GGMGDDTLD

SEQ ID NO: 10234 - protein, 9 aa, synthetic construct
GGLGNDNLT

SEQ ID NO: 10235 - protein, 9 aa, synthetic construct
GGIGADSLV

SEQ ID NO: 10236 - protein, 9 aa, synthetic construct
GGGGADTVY

SEQ ID NO: 10237 - protein, 9 aa, synthetic construct
GGLGADVML

SEQ ID NO: 10238 - protein, 9 aa, synthetic construct
GGTGRDTLR

SEQ ID NO: 10239 - protein, 9 aa, synthetic construct
GGDGSDSLY

SEQ ID NO: 10240 - protein, 9 aa, synthetic construct
GGNGADFIE

SEQ ID NO: 10241 - protein, 9 aa, synthetic construct
GGDGADFLD

SEQ ID NO: 10242 - protein, 9 aa, synthetic construct
GGYGDDLIY

SEQ ID NO: 10243 - protein, 9 aa, synthetic construct
GGAGDDYLG

SEQ ID NO: 10244 - protein, 9 aa, synthetic construct
GGGGKDTLN

SEQ ID NO: 10245 - protein, 9 aa, synthetic construct
GGTGRDVLY

SEQ ID NO: 10246 - protein, 9 aa, synthetic construct
GGEGNDSYV

SEQ ID NO: 10247 - protein, 9 aa, synthetic construct
GGRGDDTLV

SEQ ID NO: 10248 - protein, 9 aa, synthetic construct
GGIGADSLY

SEQ ID NO: 10249 - protein, 9 aa, synthetic construct
GGDGADFID

SEQ ID NO: 10250 - protein, 9 aa, synthetic construct
GGDGYDLLD

SEQ ID NO: 10251 - protein, 9 aa, synthetic construct
GGAGDDYIH

SEQ ID NO: 10252 - protein, 9 aa, synthetic construct
GGRGDDTIY

SEQ ID NO: 10253 - protein, 9 aa, synthetic construct
GGYGDDILE

SEQ ID NO: 10254 - protein, 9 aa, synthetic construct
GGLGADVMN

SEQ ID NO: 10255 - protein, 9 aa, synthetic construct
GGTGSDALY

SEQ ID NO: 10256 - protein, 9 aa, synthetic construct
GGRGDDTFV

SEQ ID NO: 10257 - protein, 9 aa, synthetic construct
GGEGSDVLT

SEQ ID NO: 10258 - protein, 9 aa, synthetic construct
GGRGDDVLT

SEQ ID NO: 10259 - protein, 9 aa, synthetic construct
GGRGDDVLV

SEQ ID NO: 10260 - protein, 9 aa, synthetic construct
GGNGVDTLT

SEQ ID NO: 10261 - protein, 9 aa, synthetic construct
GGLGADVLH

SEQ ID NO: 10262 - protein, 9 aa, synthetic construct
GGGGADLLA

SEQ ID NO: 10263 - protein, 9 aa, synthetic construct
GGEGDDALL

SEQ ID NO: 10264 - protein, 9 aa, synthetic construct
GGGGADLLE

SEQ ID NO: 10265 - protein, 9 aa, synthetic construct
GGLGRDRLT

SEQ ID NO: 10266 - protein, 9 aa, synthetic construct
GGAGRDKLF

SEQ ID NO: 10267 - protein, 9 aa, synthetic construct
GGAGEDCFC

SEQ ID NO: 10268 - protein, 9 aa, synthetic construct
GGEGNDSVF

SEQ ID NO: 10269 - protein, 9 aa, synthetic construct
GGGGDDVMI

SEQ ID NO: 10270 - protein, 9 aa, synthetic construct
GGAGEDALH

SEQ ID NO: 10271 - protein, 9 aa, synthetic construct
GGDGNDEAH

SEQ ID NO: 10272 - protein, 9 aa, synthetic construct
GGEGNDSVS

SEQ ID NO: 10273 - protein, 9 aa, synthetic construct
GGNGHDTLL

SEQ ID NO: 10274 - protein, 9 aa, synthetic construct
GGGGQDVLI

SEQ ID NO: 10275 - protein, 9 aa, synthetic construct
GGLGNDRID

SEQ ID NO: 10276 - protein, 9 aa, synthetic construct
GGAGDDYYV

SEQ ID NO: 10277 - protein, 9 aa, synthetic construct
GGTGRDTAS

SEQ ID NO: 10278 - protein, 9 aa, synthetic construct
GGAGRDLIQ

SEQ ID NO: 10279 - protein, 9 aa, synthetic construct
GGEGSDVYQ

SEQ ID NO: 10280 - protein, 9 aa, synthetic construct
GGAGRDLLE

SEQ ID NO: 10281 - protein, 9 aa, synthetic construct
GGDGADELS

SEQ ID NO: 10282 - protein, 9 aa, synthetic construct
GGRGDDSLY

SEQ ID NO: 10283 - protein, 9 aa, synthetic construct
GGDGGDRLF

SEQ ID NO: 10284 - protein, 9 aa, synthetic construct
GGGGFDTLI

SEQ ID NO: 10285 - protein, 9 aa, synthetic construct
GGRGDDLMD

SEQ ID NO: 10286 - protein, 9 aa, synthetic construct
GGAGDDVVY

SEQ ID NO: 10287 - protein, 9 aa, synthetic construct
GGEGGDTLV

SEQ ID NO: 10288 - protein, 9 aa, synthetic construct
GGLGNDQLL

SEQ ID NO: 10289 - protein, 9 aa, synthetic construct
GGLGRDRLD

SEQ ID NO: 10290 - protein, 9 aa, synthetic construct
GGRGDDKLF

SEQ ID NO: 10291 - protein, 9 aa, synthetic construct
GGDGDDEVR

SEQ ID NO: 10292 - protein, 9 aa, synthetic construct
GGAGDDVVA

SEQ ID NO: 10293 - protein, 9 aa, synthetic construct
GGRGDDILR

SEQ ID NO: 10294 - protein, 9 aa, synthetic construct
GGAGDDVMR

SEQ ID NO: 10295 - protein, 9 aa, synthetic construct
GGNGYDMLW

SEQ ID NO: 10296 - protein, 9 aa, synthetic construct
GGAGDDVMI

SEQ ID NO: 10297 - protein, 9 aa, synthetic construct
GGAGADLMD

SEQ ID NO: 10298 - protein, 9 aa, synthetic construct
GGDGEDLLY

SEQ ID NO: 10299 - protein, 9 aa, synthetic construct
GGGGDDVIR

SEQ ID NO: 10300 - protein, 9 aa, synthetic construct
GGGGADNLI

SEQ ID NO: 10301 - protein, 9 aa, synthetic construct
GGRGDDHLT

SEQ ID NO: 10302 - protein, 9 aa, synthetic construct
GGNGHDYLN

SEQ ID NO: 10303 - protein, 9 aa, synthetic construct
GGYGADYLS

SEQ ID NO: 10304 - protein, 9 aa, synthetic construct
GGLGNDQLQ

SEQ ID NO: 10305 - protein, 9 aa, synthetic construct
GGDGNDAYY

SEQ ID NO: 10306 - protein, 9 aa, synthetic construct
GGAGADLIY

SEQ ID NO: 10307 - protein, 9 aa, synthetic construct
GGDGSDTIF

SEQ ID NO: 10308 - protein, 9 aa, synthetic construct
GGDGNDDLQ

SEQ ID NO: 10309 - protein, 9 aa, synthetic construct
GGRGDDSID

SEQ ID NO: 10310 - protein, 9 aa, synthetic construct
GGDGADELH

SEQ ID NO: 10311 - protein, 9 aa, synthetic construct
GGNGHDVID

SEQ ID NO: 10312 - protein, 9 aa, synthetic construct
GGAGRDMLT

SEQ ID NO: 10313 - protein, 9 aa, synthetic construct
GGNGHDVIE

SEQ ID NO: 10314 - protein, 9 aa, synthetic construct
GGAGDDWLN

SEQ ID NO: 10315 - protein, 9 aa, synthetic construct
GGTGSDGMT

SEQ ID NO: 10316 - protein, 9 aa, synthetic construct
GGRGDDRLR

SEQ ID NO: 10317 - protein, 9 aa, synthetic construct
GGDGGDRLI

SEQ ID NO: 10318 - protein, 9 aa, synthetic construct
GGNGADDID

SEQ ID NO: 10319 - protein, 9 aa, synthetic construct
GGTGSDHLY

SEQ ID NO: 10320 - protein, 9 aa, synthetic construct
GGRGDDRIF

SEQ ID NO: 10321 - protein, 9 aa, synthetic construct
GGIGADTLQ

SEQ ID NO: 10322 - protein, 9 aa, synthetic construct
GGTGSDILN

SEQ ID NO: 10323 - protein, 9 aa, synthetic construct
GGTGSDILV

SEQ ID NO: 10324 - protein, 9 aa, synthetic construct
GGLGDDAID

SEQ ID NO: 10325 - protein, 9 aa, synthetic construct
GGDGNDDID

SEQ ID NO: 10326 - protein, 9 aa, synthetic construct
GGAGADLLG

SEQ ID NO: 10327 - protein, 9 aa, synthetic construct
GGGGHDRLR

SEQ ID NO: 10328 - protein, 9 aa, synthetic construct
GGAGYDTLD

SEQ ID NO: 10329 - protein, 9 aa, synthetic construct
GGGGVDHLY

SEQ ID NO: 10330 - protein, 9 aa, synthetic construct
GGAGSDLIR

SEQ ID NO: 10331 - protein, 9 aa, synthetic construct
GGVGADTMY

SEQ ID NO: 10332 - protein, 9 aa, synthetic construct
GGAGSDLFL

SEQ ID NO: 10333 - protein, 9 aa, synthetic construct
GGGGRDILR

SEQ ID NO: 10334 - protein, 9 aa, synthetic construct
GGEGSDSLM

SEQ ID NO: 10335 - protein, 9 aa, synthetic construct
GGEGADQMA

SEQ ID NO: 10336 - protein, 9 aa, synthetic construct
GGVGADVLI

SEQ ID NO: 10337 - protein, 9 aa, synthetic construct
GGDGHDTIS

SEQ ID NO: 10338 - protein, 9 aa, synthetic construct
GGLGNDHLS

SEQ ID NO: 10339 - protein, 9 aa, synthetic construct
GGAGDDNLV

SEQ ID NO: 10340 - protein, 9 aa, synthetic construct
GGVGADVLT

SEQ ID NO: 10341 - protein, 9 aa, synthetic construct
GGIGADLFI

SEQ ID NO: 10342 - protein, 9 aa, synthetic construct
GGPGDDTLH

SEQ ID NO: 10343 - protein, 9 aa, synthetic construct
GGLGNDHLE

SEQ ID NO: 10344 - protein, 9 aa, synthetic construct
GGAGADRLK

SEQ ID NO: 10345 - protein, 9 aa, synthetic construct
GGQGNDSLI

SEQ ID NO: 10346 - protein, 9 aa, synthetic construct
GGAGDDNLG

SEQ ID NO: 10347 - protein, 9 aa, synthetic construct
GGDGTDHLV

SEQ ID NO: 10348 - protein, 9 aa, synthetic construct
GGQGNDSIA

SEQ ID NO: 10349 - protein, 9 aa, synthetic construct
GGEGSDSLD

SEQ ID NO: 10350 - protein, 9 aa, synthetic construct
GGAGSDLLK

SEQ ID NO: 10351 - protein, 9 aa, synthetic construct
GGQGNDTIN

SEQ ID NO: 10352 - protein, 9 aa, synthetic construct
GGQGNDTIS

SEQ ID NO: 10353 - protein, 9 aa, synthetic construct
GGDGHDTIH

SEQ ID NO: 10354 - protein, 9 aa, synthetic construct
GGPGDDSMG

SEQ ID NO: 10355 - protein, 9 aa, synthetic construct
GGLGDDRYI

SEQ ID NO: 10356 - protein, 9 aa, synthetic construct
GGGGADTIR

SEQ ID NO: 10357 - protein, 9 aa, synthetic construct
GGLGDDRYV

SEQ ID NO: 10358 - protein, 9 aa, synthetic construct
GGVGADRLI

SEQ ID NO: 10359 - protein, 9 aa, synthetic construct
GGVGADRLT

SEQ ID NO: 10360 - protein, 9 aa, synthetic construct
GGGGVDRLS

SEQ ID NO: 10361 - protein, 9 aa, synthetic construct
GGDGLDTLN

SEQ ID NO: 10362 - protein, 9 aa, synthetic construct
GGGGRDIFV

SEQ ID NO: 10363 - protein, 9 aa, synthetic construct
GGQGNDVID

SEQ ID NO: 10364 - protein, 9 aa, synthetic construct
GGQGNDTYY

SEQ ID NO: 10365 - protein, 9 aa, synthetic construct
GGLGDDSID

SEQ ID NO: 10366 - protein, 9 aa, synthetic construct
GGQGNDTYL

SEQ ID NO: 10367 - protein, 9 aa, synthetic construct
GGPGDDRLT

SEQ ID NO: 10368 - protein, 9 aa, synthetic construct
GGAGDDQIN

SEQ ID NO: 10369 - protein, 9 aa, synthetic construct
GGHGSDEIY

SEQ ID NO: 10370 - protein, 9 aa, synthetic construct
GGDGHDALY

SEQ ID NO: 10371 - protein, 9 aa, synthetic construct
GGVGADTIT

SEQ ID NO: 10372 - protein, 9 aa, synthetic construct
GGEGDDLIR

SEQ ID NO: 10373 - protein, 9 aa, synthetic construct
GGVGADTLR

SEQ ID NO: 10374 - protein, 9 aa, synthetic construct
GGEGSDSIL

SEQ ID NO: 10375 - protein, 9 aa, synthetic construct
GGGGRDKLF

SEQ ID NO: 10376 - protein, 9 aa, synthetic construct
GGAGDDNID

SEQ ID NO: 10377 - protein, 9 aa, synthetic construct
GGVGDDILS

SEQ ID NO: 10378 - protein, 9 aa, synthetic construct
GGQGNDLLL

SEQ ID NO: 10379 - protein, 9 aa, synthetic construct
GGQGNDLLI

SEQ ID NO: 10380 - protein, 9 aa, synthetic construct
GGAGSDMLL

SEQ ID NO: 10381 - protein, 9 aa, synthetic construct
GGQGNDLLF

SEQ ID NO: 10382 - protein, 9 aa, synthetic construct
GGLGDDTFY

SEQ ID NO: 10383 - protein, 9 aa, synthetic construct
GGAGDDMIG

SEQ ID NO: 10384 - protein, 9 aa, synthetic construct
GGGGDDRLH

SEQ ID NO: 10385 - protein, 9 aa, synthetic construct
GGAGDDMIA

SEQ ID NO: 10386 - protein, 9 aa, synthetic construct
GGAGSDMLW

SEQ ID NO: 10387 - protein, 9 aa, synthetic construct
GGDGHDTLM

SEQ ID NO: 10388 - protein, 9 aa, synthetic construct
GGLGNDFLV

SEQ ID NO: 10389 - protein, 9 aa, synthetic construct
GGVGDDLLY

SEQ ID NO: 10390 - protein, 9 aa, synthetic construct
GGLGDDTLG

SEQ ID NO: 10391 - protein, 9 aa, synthetic construct
GGLGDDTLH

SEQ ID NO: 10392 - protein, 9 aa, synthetic construct
GGMGNDYLY

SEQ ID NO: 10393 - protein, 9 aa, synthetic construct
GGVGDDMLD

SEQ ID NO: 10394 - protein, 9 aa, synthetic construct
GGAGDDLVN

SEQ ID NO: 10395 - protein, 9 aa, synthetic construct
GGAGDDLVD

SEQ ID NO: 10396 - protein, 9 aa, synthetic construct
GGLGDDTMD

SEQ ID NO: 10397 - protein, 9 aa, synthetic construct
GGPGDDVLW

SEQ ID NO: 10398 - protein, 9 aa, synthetic construct
GGAGDDMLE

SEQ ID NO: 10399 - protein, 9 aa, synthetic construct
GGQGNDRLI

SEQ ID NO: 10400 - protein, 9 aa, synthetic construct
GGAGSDMLF

SEQ ID NO: 10401 - protein, 9 aa, synthetic construct
GGGGRDKLI

SEQ ID NO: 10402 - protein, 9 aa, synthetic construct
GGAGDDNIA

SEQ ID NO: 10403 - protein, 9 aa, synthetic construct
GGDGLDTLF

SEQ ID NO: 10404 - protein, 9 aa, synthetic construct
GGPGDDTYT

SEQ ID NO: 10405 - protein, 9 aa, synthetic construct
GGDGLDTLD

SEQ ID NO: 10406 - protein, 9 aa, synthetic construct
GGAGSDLLY

SEQ ID NO: 10407 - protein, 9 aa, synthetic construct
GGDGTDILI

SEQ ID NO: 10408 - protein, 9 aa, synthetic construct
GGDGTDILN

SEQ ID NO: 10409 - protein, 9 aa, synthetic construct
GGDGGDTFV

SEQ ID NO: 10410 - protein, 9 aa, synthetic construct
GGDGLDTAV

SEQ ID NO: 10411 - protein, 9 aa, synthetic construct
GGGGVDTAS

SEQ ID NO: 10412 - protein, 9 aa, synthetic construct
GGNGNDLVD

SEQ ID NO: 10413 - protein, 9 aa, synthetic construct
GGDGLDTAD

SEQ ID NO: 10414 - protein, 9 aa, synthetic construct
GGVGDDIIT

SEQ ID NO: 10415 - protein, 9 aa, synthetic construct
GGGGADTMS

SEQ ID NO: 10416 - protein, 9 aa, synthetic construct
GGEGRDSLT

SEQ ID NO: 10417 - protein, 9 aa, synthetic construct
GGDGEDVLN

SEQ ID NO: 10418 - protein, 9 aa, synthetic construct
GGLGDDTFL

SEQ ID NO: 10419 - protein, 9 aa, synthetic construct
GGQGNDLVD

SEQ ID NO: 10420 - protein, 9 aa, synthetic construct
GGQGNDWLS

SEQ ID NO: 10421 - protein, 9 aa, synthetic construct
GGWGNDTID

SEQ ID NO: 10422 - protein, 9 aa, synthetic construct
GGGGDDSLE

SEQ ID NO: 10423 - protein, 9 aa, synthetic construct
GGAGSDAIT

SEQ ID NO: 10424 - protein, 9 aa, synthetic construct
GGTGVDSMT

SEQ ID NO: 10425 - protein, 9 aa, synthetic construct
GGTGVDTAT

SEQ ID NO: 10426 - protein, 9 aa, synthetic construct
GGAGSDALS

SEQ ID NO: 10427 - protein, 9 aa, synthetic construct
GGLGNDLFR

SEQ ID NO: 10428 - protein, 9 aa, synthetic construct
GGDGFDILY

SEQ ID NO: 10429 - protein, 9 aa, synthetic construct
GGTGVDTLD

SEQ ID NO: 10430 - protein, 9 aa, synthetic construct
GGPGDDFLY

SEQ ID NO: 10431 - protein, 9 aa, synthetic construct
GGEGDDIYV

SEQ ID NO: 10432 - protein, 9 aa, synthetic construct
GGEGDDDIF

SEQ ID NO: 10433 - protein, 9 aa, synthetic construct
GGQGSDTLN

SEQ ID NO: 10434 - protein, 9 aa, synthetic construct
GGQGSDTLM

SEQ ID NO: 10435 - protein, 9 aa, synthetic construct
GGEGRDRLF

SEQ ID NO: 10436 - protein, 9 aa, synthetic construct
GGDGSDVLN

SEQ ID NO: 10437 - protein, 9 aa, synthetic construct
GGLGTDVAL

SEQ ID NO: 10438 - protein, 9 aa, synthetic construct
GGEGADKLY

SEQ ID NO: 10439 - protein, 9 aa, synthetic construct
GGWGSDALF

SEQ ID NO: 10440 - protein, 9 aa, synthetic construct
GGQGSDSLD

SEQ ID NO: 10441 - protein, 9 aa, synthetic construct
GGAGADQLA

SEQ ID NO: 10442 - protein, 9 aa, synthetic construct
GGLGNDKLA

SEQ ID NO: 10443 - protein, 9 aa, synthetic construct
GGTGVDSAS

SEQ ID NO: 10444 - protein, 9 aa, synthetic construct
GGAGSDAFV

SEQ ID NO: 10445 - protein, 9 aa, synthetic construct
GGAGDDRYI

SEQ ID NO: 10446 - protein, 9 aa, synthetic construct
GGAGRDYLY

SEQ ID NO: 10447 - protein, 9 aa, synthetic construct
GGAGRDVMY

SEQ ID NO: 10448 - protein, 9 aa, synthetic construct
GGQGVDTLI

SEQ ID NO: 10449 - protein, 9 aa, synthetic construct
GGLGNDLIE

SEQ ID NO: 10450 - protein, 9 aa, synthetic construct
GGAGDDSYY

SEQ ID NO: 10451 - protein, 9 aa, synthetic construct
GGGGDDTIF

SEQ ID NO: 10452 - protein, 9 aa, synthetic construct
GGQGVDSLT

SEQ ID NO: 10453 - protein, 9 aa, synthetic construct
GGEGSDTVA

SEQ ID NO: 10454 - protein, 9 aa, synthetic construct
GGAGRDWLE

SEQ ID NO: 10455 - protein, 9 aa, synthetic construct
GGTGVDELT

SEQ ID NO: 10456 - protein, 9 aa, synthetic construct
GGAGDDSVT

SEQ ID NO: 10457 - protein, 9 aa, synthetic construct
GGGGDDTIA

SEQ ID NO: 10458 - protein, 9 aa, synthetic construct
GGAGYDRMT

SEQ ID NO: 10459 - protein, 9 aa, synthetic construct
GGAGDDSVD

SEQ ID NO: 10460 - protein, 9 aa, synthetic construct
GGLGDDLIF

SEQ ID NO: 10461 - protein, 9 aa, synthetic construct
GGIGADILT

SEQ ID NO: 10462 - protein, 9 aa, synthetic construct
GGEGSDTLS

SEQ ID NO: 10463 - protein, 9 aa, synthetic construct
GGIGADILQ

SEQ ID NO: 10464 - protein, 9 aa, synthetic construct
GGAGYDRLW

SEQ ID NO: 10465 - protein, 9 aa, synthetic construct
GGDGSDVIY

SEQ ID NO: 10466 - protein, 9 aa, synthetic construct
GGGGRDELD

SEQ ID NO: 10467 - protein, 9 aa, synthetic construct
GGGGADSIN

SEQ ID NO: 10468 - protein, 9 aa, synthetic construct
GGDGADVLE

SEQ ID NO: 10469 - protein, 9 aa, synthetic construct
GGLGDDQLR

SEQ ID NO: 10470 - protein, 9 aa, synthetic construct
GGVGADILN

SEQ ID NO: 10471 - protein, 9 aa, synthetic construct
GGVGADILS

SEQ ID NO: 10472 - protein, 9 aa, synthetic construct
GGQGQDWME

SEQ ID NO: 10473 - protein, 9 aa, synthetic construct
GGAGADQMI

SEQ ID NO: 10474 - protein, 9 aa, synthetic construct
GGLGDDRID

SEQ ID NO: 10475 - protein, 9 aa, synthetic construct
GGWGNDTLS

SEQ ID NO: 10476 - protein, 9 aa, synthetic construct
GGQGQDTIH

SEQ ID NO: 10477 - protein, 9 aa, synthetic construct
GGVGADKMT

SEQ ID NO: 10478 - protein, 9 aa, synthetic construct
GGLGDDRIE

SEQ ID NO: 10479 - protein, 9 aa, synthetic construct
GGGGNDFMD

SEQ ID NO: 10480 - protein, 9 aa, synthetic construct
GGHGSDYIE

SEQ ID NO: 10481 - protein, 9 aa, synthetic construct
GGAGDDQMT

SEQ ID NO: 10482 - protein, 9 aa, synthetic construct
GGAGSDIIS

SEQ ID NO: 10483 - protein, 9 aa, synthetic construct
GGAGSDIIY

SEQ ID NO: 10484 - protein, 9 aa, synthetic construct
GGAGSDILQ

SEQ ID NO: 10485 - protein, 9 aa, synthetic construct
GGDGSDYLY

SEQ ID NO: 10486 - protein, 9 aa, synthetic construct
GGGGADTIH

SEQ ID NO: 10487 - protein, 9 aa, synthetic construct
GGMGDDVLT

SEQ ID NO: 10488 - protein, 9 aa, synthetic construct
GGLGVDALN

SEQ ID NO: 10489 - protein, 9 aa, synthetic construct
GGDGHDSLW

SEQ ID NO: 10490 - protein, 9 aa, synthetic construct
GGEGNDTIK

SEQ ID NO: 10491 - protein, 9 aa, synthetic construct
GGEGSDTIF

SEQ ID NO: 10492 - protein, 9 aa, synthetic construct
GGLGDDQLI

SEQ ID NO: 10493 - protein, 9 aa, synthetic construct
GGAGDDRMT

SEQ ID NO: 10494 - protein, 9 aa, synthetic construct
GGAGSDELS

SEQ ID NO: 10495 - protein, 9 aa, synthetic construct
GGEGSDTIE

SEQ ID NO: 10496 - protein, 9 aa, synthetic construct
GGLGDDNIG

SEQ ID NO: 10497 - protein, 9 aa, synthetic construct
GGLGNDKIY

SEQ ID NO: 10498 - protein, 9 aa, synthetic construct
GGGGADSLL

SEQ ID NO: 10499 - protein, 9 aa, synthetic construct
GGAGDDRLK

SEQ ID NO: 10500 - protein, 9 aa, synthetic construct
GGDGLDWAV

SEQ ID NO: 10501 - protein, 9 aa, synthetic construct
GGLGDDNLQ

SEQ ID NO: 10502 - protein, 9 aa, synthetic construct
GGAGDDRLH

SEQ ID NO: 10503 - protein, 9 aa, synthetic construct
GGQGRDTYV

SEQ ID NO: 10504 - protein, 9 aa, synthetic construct
GGAGADQLQ

SEQ ID NO: 10505 - protein, 9 aa, synthetic construct
GGAGDDRIY

SEQ ID NO: 10506 - protein, 9 aa, synthetic construct
GGAGSDFLA

SEQ ID NO: 10507 - protein, 9 aa, synthetic construct
GGPGDDIMY

SEQ ID NO: 10508 - protein, 9 aa, synthetic construct
GGGGADSMS

SEQ ID NO: 10509 - protein, 9 aa, synthetic construct
GGNGNDNIS

SEQ ID NO: 10510 - protein, 9 aa, synthetic construct
GGEGEDILD

SEQ ID NO: 10511 - protein, 9 aa, synthetic construct
GGEGSDTFL

SEQ ID NO: 10512 - protein, 9 aa, synthetic construct
GGEGLDYLW

SEQ ID NO: 10513 - protein, 9 aa, synthetic construct
GGDGSDSIE

SEQ ID NO: 10514 - protein, 9 aa, synthetic construct
GGAGNDFLG

SEQ ID NO: 10515 - protein, 9 aa, synthetic construct
GGSGIDQLK

SEQ ID NO: 10516 - protein, 9 aa, synthetic construct
GGDGNDTVA

SEQ ID NO: 10517 - protein, 9 aa, synthetic construct
GGKGLDIMV

SEQ ID NO: 10518 - protein, 9 aa, synthetic construct
GGIGSDTFV

SEQ ID NO: 10519 - protein, 9 aa, synthetic construct
GGIGRDTLD

SEQ ID NO: 10520 - protein, 9 aa, synthetic construct
GGAGLDTLA

SEQ ID NO: 10521 - protein, 9 aa, synthetic construct
GGSGNDVII

SEQ ID NO: 10522 - protein, 9 aa, synthetic construct
GGAGKDFLS

SEQ ID NO: 10523 - protein, 9 aa, synthetic construct
GGAGLDTLE

SEQ ID NO: 10524 - protein, 9 aa, synthetic construct
GGAGLDALY

SEQ ID NO: 10525 - protein, 9 aa, synthetic construct
GGGGNDRLH

SEQ ID NO: 10526 - protein, 9 aa, synthetic construct
GGGGNDTLG

SEQ ID NO: 10527 - protein, 9 aa, synthetic construct
GGKGADQLV

SEQ ID NO: 10528 - protein, 9 aa, synthetic construct
GGDGDDQLA

SEQ ID NO: 10529 - protein, 9 aa, synthetic construct
GGKGDDMLL

SEQ ID NO: 10530 - protein, 9 aa, synthetic construct
GGSGNDRLK

SEQ ID NO: 10531 - protein, 9 aa, synthetic construct
GGSGNDRLH

SEQ ID NO: 10532 - protein, 9 aa, synthetic construct
GGAGKDMLT

SEQ ID NO: 10533 - protein, 9 aa, synthetic construct
GGSGTDLIY

SEQ ID NO: 10534 - protein, 9 aa, synthetic construct
GGNGDDSID

SEQ ID NO: 10535 - protein, 9 aa, synthetic construct
GGAGKDFII

SEQ ID NO: 10536 - protein, 9 aa, synthetic construct
GGAGKDFID

SEQ ID NO: 10537 - protein, 9 aa, synthetic construct
GGSGNDRIW

SEQ ID NO: 10538 - protein, 9 aa, synthetic construct
GGSGNDRIV

SEQ ID NO: 10539 - protein, 9 aa, synthetic construct
GGSGNDRIT

SEQ ID NO: 10540 - protein, 9 aa, synthetic construct
GGSGNDIFV

SEQ ID NO: 10541 - protein, 9 aa, synthetic construct
GGSGNDRIS

SEQ ID NO: 10542 - protein, 9 aa, synthetic construct
GGNGDDSLS

SEQ ID NO: 10543 - protein, 9 aa, synthetic construct
GGSGGDTYL

SEQ ID NO: 10544 - protein, 9 aa, synthetic construct
GGSGNDIID

SEQ ID NO: 10545 - protein, 9 aa, synthetic construct
GGSGSDMVF

SEQ ID NO: 10546 - protein, 9 aa, synthetic construct
GGAGKDNLQ

SEQ ID NO: 10547 - protein, 9 aa, synthetic construct
GGKGNDGYG

SEQ ID NO: 10548 - protein, 9 aa, synthetic construct
GGSGNDVFS

SEQ ID NO: 10549 - protein, 9 aa, synthetic construct
GGAGHDTID

SEQ ID NO: 10550 - protein, 9 aa, synthetic construct
GGDGNDSLG

SEQ ID NO: 10551 - protein, 9 aa, synthetic construct
GGTGADIFD

SEQ ID NO: 10552 - protein, 9 aa, synthetic construct
GGTGADRIF

SEQ ID NO: 10553 - protein, 9 aa, synthetic construct
GGSGNDGLT

SEQ ID NO: 10554 - protein, 9 aa, synthetic construct
GGEGADVLI

SEQ ID NO: 10555 - protein, 9 aa, synthetic construct
GGSGQDYLL

SEQ ID NO: 10556 - protein, 9 aa, synthetic construct
GGAGKDIFR

SEQ ID NO: 10557 - protein, 9 aa, synthetic construct
GGGGNDTIM

SEQ ID NO: 10558 - protein, 9 aa, synthetic construct
GGTGADIIY

SEQ ID NO: 10559 - protein, 9 aa, synthetic construct
GGSGNDTYR

SEQ ID NO: 10560 - protein, 9 aa, synthetic construct
GGKGHDIIV

SEQ ID NO: 10561 - protein, 9 aa, synthetic construct
GGAGIDLIS

SEQ ID NO: 10562 - protein, 9 aa, synthetic construct
GGKGDDNLY

SEQ ID NO: 10563 - protein, 9 aa, synthetic construct
GGAGNDIYA

SEQ ID NO: 10564 - protein, 9 aa, synthetic construct
GGIGTDQLS

SEQ ID NO: 10565 - protein, 9 aa, synthetic construct
GGKGDDTII

SEQ ID NO: 10566 - protein, 9 aa, synthetic construct
GGFGFDRMN

SEQ ID NO: 10567 - protein, 9 aa, synthetic construct
GGDGNDTVR

SEQ ID NO: 10568 - protein, 9 aa, synthetic construct
GGAGKDIFI

SEQ ID NO: 10569 - protein, 9 aa, synthetic construct
GGSGQDYMN

SEQ ID NO: 10570 - protein, 9 aa, synthetic construct
GGKGDDVLW

SEQ ID NO: 10571 - protein, 9 aa, synthetic construct
GGTGADRFL

SEQ ID NO: 10572 - protein, 9 aa, synthetic construct
GGKGADTMT

SEQ ID NO: 10573 - protein, 9 aa, synthetic construct
GGDGDDLAY

SEQ ID NO: 10574 - protein, 9 aa, synthetic construct
GGSGNDHIS

SEQ ID NO: 10575 - protein, 9 aa, synthetic construct
GGIGRDTLS

SEQ ID NO: 10576 - protein, 9 aa, synthetic construct
GGKGDDVLR

SEQ ID NO: 10577 - protein, 9 aa, synthetic construct
GGDGNDTVK

SEQ ID NO: 10578 - protein, 9 aa, synthetic construct
GGFGLDVIQ

SEQ ID NO: 10579 - protein, 9 aa, synthetic construct
GGSGNDHLF

SEQ ID NO: 10580 - protein, 9 aa, synthetic construct
GGDGDDMII

SEQ ID NO: 10581 - protein, 9 aa, synthetic construct
GGSGNDHLR

SEQ ID NO: 10582 - protein, 9 aa, synthetic construct
GGSGNDRIN

SEQ ID NO: 10583 - protein, 9 aa, synthetic construct
GGTGDDALT

SEQ ID NO: 10584 - protein, 9 aa, synthetic construct
GGDGNDVMS

SEQ ID NO: 10585 - protein, 9 aa, synthetic construct
GGSGNDIYV

SEQ ID NO: 10586 - protein, 9 aa, synthetic construct
GGTGADKMA

SEQ ID NO: 10587 - protein, 9 aa, synthetic construct
GGKGDDVLE

SEQ ID NO: 10588 - protein, 9 aa, synthetic construct
GGNGDDLID

SEQ ID NO: 10589 - protein, 9 aa, synthetic construct
GGSGPDMFL

SEQ ID NO: 10590 - protein, 9 aa, synthetic construct
GGDGDDLFI

SEQ ID NO: 10591 - protein, 9 aa, synthetic construct
GGSGSDLLN

SEQ ID NO: 10592 - protein, 9 aa, synthetic construct
GGAGKDSFV

SEQ ID NO: 10593 - protein, 9 aa, synthetic construct
GGFGDDMLS

SEQ ID NO: 10594 - protein, 9 aa, synthetic construct
GGTGDDEIH

SEQ ID NO: 10595 - protein, 9 aa, synthetic construct
GGTGADKLI

SEQ ID NO: 10596 - protein, 9 aa, synthetic construct
GGSGSDLLQ

SEQ ID NO: 10597 - protein, 9 aa, synthetic construct
GGKGGDRLW

SEQ ID NO: 10598 - protein, 9 aa, synthetic construct
GGFGEDVLR

SEQ ID NO: 10599 - protein, 9 aa, synthetic construct
GGAGIDKLD

SEQ ID NO: 10600 - protein, 9 aa, synthetic construct
GGSGNDKIT

SEQ ID NO: 10601 - protein, 9 aa, synthetic construct
GGSGNDKIY

SEQ ID NO: 10602 - protein, 9 aa, synthetic construct
GGSGGDSLA

SEQ ID NO: 10603 - protein, 9 aa, synthetic construct
GGGGNDTYL

SEQ ID NO: 10604 - protein, 9 aa, synthetic construct
GGNGDDELY

SEQ ID NO: 10605 - protein, 9 aa, synthetic construct
GGNGDDRLH

SEQ ID NO: 10606 - protein, 9 aa, synthetic construct
GGAGNDEMS

SEQ ID NO: 10607 - protein, 9 aa, synthetic construct
GGAGKDYID

SEQ ID NO: 10608 - protein, 9 aa, synthetic construct
GGSGNDQMK

SEQ ID NO: 10609 - protein, 9 aa, synthetic construct
GGEGNDAIN

SEQ ID NO: 10610 - protein, 9 aa, synthetic construct
GGEGADVLY

SEQ ID NO: 10611 - protein, 9 aa, synthetic construct
GGLGSDLYI

SEQ ID NO: 10612 - protein, 9 aa, synthetic construct
GGSGRDRLS

SEQ ID NO: 10613 - protein, 9 aa, synthetic construct
GGSGNDVVA

SEQ ID NO: 10614 - protein, 9 aa, synthetic construct
GGKGDDTLR

SEQ ID NO: 10615 - protein, 9 aa, synthetic construct
GGFGDDVLT

SEQ ID NO: 10616 - protein, 9 aa, synthetic construct
GGAGMDRLY

SEQ ID NO: 10617 - protein, 9 aa, synthetic construct
GGDGNDTMR

SEQ ID NO: 10618 - protein, 9 aa, synthetic construct
GGTGDDDLV

SEQ ID NO: 10619 - protein, 9 aa, synthetic construct
GGSGKDTLL

SEQ ID NO: 10620 - protein, 9 aa, synthetic construct
GGSGGDTLE

SEQ ID NO: 10621 - protein, 9 aa, synthetic construct
GGSGNDIIH

SEQ ID NO: 10622 - protein, 9 aa, synthetic construct
GGTGADQLW

SEQ ID NO: 10623 - protein, 9 aa, synthetic construct
GGKGGDTID

SEQ ID NO: 10624 - protein, 9 aa, synthetic construct
GGDGDDNLN

SEQ ID NO: 10625 - protein, 9 aa, synthetic construct
GGAGNDKIL

SEQ ID NO: 10626 - protein, 9 aa, synthetic construct
GGFGLDTLD

SEQ ID NO: 10627 - protein, 9 aa, synthetic construct
GGSGSDELT

SEQ ID NO: 10628 - protein, 9 aa, synthetic construct
GGDGDDNLQ

SEQ ID NO: 10629 - protein, 9 aa, synthetic construct
GGSGVDTIS

SEQ ID NO: 10630 - protein, 9 aa, synthetic construct
GGDGDDQLH

SEQ ID NO: 10631 - protein, 9 aa, synthetic construct
GGAGNDGLA

SEQ ID NO: 10632 - protein, 9 aa, synthetic construct
GGTGADIMA

SEQ ID NO: 10633 - protein, 9 aa, synthetic construct
GGKGADELR

SEQ ID NO: 10634 - protein, 9 aa, synthetic construct
GGSGKDTLY

SEQ ID NO: 10635 - protein, 9 aa, synthetic construct
GGDGNDYIY

SEQ ID NO: 10636 - protein, 9 aa, synthetic construct
GGSGSDLLR

SEQ ID NO: 10637 - protein, 9 aa, synthetic construct
GGNGDDQLV

SEQ ID NO: 10638 - protein, 9 aa, synthetic construct
GGTGADIML

SEQ ID NO: 10639 - protein, 9 aa, synthetic construct
GGEGADTVF

SEQ ID NO: 10640 - protein, 9 aa, synthetic construct
GGSGKDTLS

SEQ ID NO: 10641 - protein, 9 aa, synthetic construct
GGAGIDKLS

SEQ ID NO: 10642 - protein, 9 aa, synthetic construct
GGKGEDTFM

SEQ ID NO: 10643 - protein, 9 aa, synthetic construct
GGKGADVLR

SEQ ID NO: 10644 - protein, 9 aa, synthetic construct
GGSGVDTAD

SEQ ID NO: 10645 - protein, 9 aa, synthetic construct
GGAGLDVLT

SEQ ID NO: 10646 - protein, 9 aa, synthetic construct
GGGGNDQIF

SEQ ID NO: 10647 - protein, 9 aa, synthetic construct
GGAGKDELY

SEQ ID NO: 10648 - protein, 9 aa, synthetic construct
GGAGKDVAL

SEQ ID NO: 10649 - protein, 9 aa, synthetic construct
GGSGSDFIE

SEQ ID NO: 10650 - protein, 9 aa, synthetic construct
GGSGIDSLY

SEQ ID NO: 10651 - protein, 9 aa, synthetic construct
GGKGADRID

SEQ ID NO: 10652 - protein, 9 aa, synthetic construct
GGGGNDQLT

SEQ ID NO: 10653 - protein, 9 aa, synthetic construct
GGTGADYLT

SEQ ID NO: 10654 - protein, 9 aa, synthetic construct
GGSGSDVLI

SEQ ID NO: 10655 - protein, 9 aa, synthetic construct
GGTGADSMS

SEQ ID NO: 10656 - protein, 9 aa, synthetic construct
GGSGHDQLT

SEQ ID NO: 10657 - protein, 9 aa, synthetic construct
GGSGQDLLR

SEQ ID NO: 10658 - protein, 9 aa, synthetic construct
GGTGADDMT

SEQ ID NO: 10659 - protein, 9 aa, synthetic construct
GGEGKDVFV

SEQ ID NO: 10660 - protein, 9 aa, synthetic construct
GGEGNDHLS

SEQ ID NO: 10661 - protein, 9 aa, synthetic construct
GGAGNDIIK

SEQ ID NO: 10662 - protein, 9 aa, synthetic construct
GGSGNDEIL

SEQ ID NO: 10663 - protein, 9 aa, synthetic construct
GGTGADTFD

SEQ ID NO: 10664 - protein, 9 aa, synthetic construct
GGEGADVID

SEQ ID NO: 10665 - protein, 9 aa, synthetic construct
GGIGTDVAS

SEQ ID NO: 10666 - protein, 9 aa, synthetic construct
GGSGHDRLA

SEQ ID NO: 10667 - protein, 9 aa, synthetic construct
GGAGNDIIG

SEQ ID NO: 10668 - protein, 9 aa, synthetic construct
GGKGDDRLY

SEQ ID NO: 10669 - protein, 9 aa, synthetic construct
GGNGDDTYF

SEQ ID NO: 10670 - protein, 9 aa, synthetic construct
GGAGNDALK

SEQ ID NO: 10671 - protein, 9 aa, synthetic construct
GGSGYDTIH

SEQ ID NO: 10672 - protein, 9 aa, synthetic construct
GGNGDDFLF

SEQ ID NO: 10673 - protein, 9 aa, synthetic construct
GGSGQDTFR

SEQ ID NO: 10674 - protein, 9 aa, synthetic construct
GGGGNDTMS

SEQ ID NO: 10675 - protein, 9 aa, synthetic construct
GGTGADVIL

SEQ ID NO: 10676 - protein, 9 aa, synthetic construct
GGAGNDALG

SEQ ID NO: 10677 - protein, 9 aa, synthetic construct
GGSGSDTIL

SEQ ID NO: 10678 - protein, 9 aa, synthetic construct
GGTGADSMN

SEQ ID NO: 10679 - protein, 9 aa, synthetic construct
GGAGKDKLT

SEQ ID NO: 10680 - protein, 9 aa, synthetic construct
GGGGGDLLR

SEQ ID NO: 10681 - protein, 9 aa, synthetic construct
GGAGNDILC

SEQ ID NO: 10682 - protein, 9 aa, synthetic construct
GGSGNDTLG

SEQ ID NO: 10683 - protein, 9 aa, synthetic construct
GGIGVDTIV

SEQ ID NO: 10684 - protein, 9 aa, synthetic construct
GGGGGDLLK

SEQ ID NO: 10685 - protein, 9 aa, synthetic construct
GGDGDDMID

SEQ ID NO: 10686 - protein, 9 aa, synthetic construct
GGSGHDTLN

SEQ ID NO: 10687 - protein, 9 aa, synthetic construct
GGIGVDSLD

SEQ ID NO: 10688 - protein, 9 aa, synthetic construct
GGDGQDLFV

SEQ ID NO: 10689 - protein, 9 aa, synthetic construct
GGSGSDTVI

SEQ ID NO: 10690 - protein, 9 aa, synthetic construct
GGGGNDRIL

SEQ ID NO: 10691 - protein, 9 aa, synthetic construct
GGIGSDILI

SEQ ID NO: 10692 - protein, 9 aa, synthetic construct
GGSGNDAIF

SEQ ID NO: 10693 - protein, 9 aa, synthetic construct
GGSGRDYLF

SEQ ID NO: 10694 - protein, 9 aa, synthetic construct
GGNGDDTIV

SEQ ID NO: 10695 - protein, 9 aa, synthetic construct
GGSGNDAIS

SEQ ID NO: 10696 - protein, 9 aa, synthetic construct
GGKGDDVYV

SEQ ID NO: 10697 - protein, 9 aa, synthetic construct
GGSGNDAIT

SEQ ID NO: 10698 - protein, 9 aa, synthetic construct
GGFGNDTLA

SEQ ID NO: 10699 - protein, 9 aa, synthetic construct
GGSGRDYLD

SEQ ID NO: 10700 - protein, 9 aa, synthetic construct
GGAGNDAYY

SEQ ID NO: 10701 - protein, 9 aa, synthetic construct
GGAGKDTFL

SEQ ID NO: 10702 - protein, 9 aa, synthetic construct
GGTGADALL

SEQ ID NO: 10703 - protein, 9 aa, synthetic construct
GGEGDDNLY

SEQ ID NO: 10704 - protein, 9 aa, synthetic construct
GGSGNDALI

SEQ ID NO: 10705 - protein, 9 aa, synthetic construct
GGKGDDGLF

SEQ ID NO: 10706 - protein, 9 aa, synthetic construct
GGEGDDNLG

SEQ ID NO: 10707 - protein, 9 aa, synthetic construct
GGDGNDTYH

SEQ ID NO: 10708 - protein, 9 aa, synthetic construct
GGSGMDTLS

SEQ ID NO: 10709 - protein, 9 aa, synthetic construct
GGSGNDSYL

SEQ ID NO: 10710 - protein, 9 aa, synthetic construct
GGFGDDTLF

SEQ ID NO: 10711 - protein, 9 aa, synthetic construct
GGIGVDLMI

SEQ ID NO: 10712 - protein, 9 aa, synthetic construct
GGAGLDILN

SEQ ID NO: 10713 - protein, 9 aa, synthetic construct
GGAGIDRAV

SEQ ID NO: 10714 - protein, 9 aa, synthetic construct
GGGGNDTFK

SEQ ID NO: 10715 - protein, 9 aa, synthetic construct
GGFGNDTIY

SEQ ID NO: 10716 - protein, 9 aa, synthetic construct
GGIGVDRLF

SEQ ID NO: 10717 - protein, 9 aa, synthetic construct
GGGGNDTFT

SEQ ID NO: 10718 - protein, 9 aa, synthetic construct
GGSGHDRLY

SEQ ID NO: 10719 - protein, 9 aa, synthetic construct
GGKGADTFL

SEQ ID NO: 10720 - protein, 9 aa, synthetic construct
GGSGHDVLD

SEQ ID NO: 10721 - protein, 9 aa, synthetic construct
GGAGNDDLQ

SEQ ID NO: 10722 - protein, 9 aa, synthetic construct
GGTGADHLA

SEQ ID NO: 10723 - protein, 9 aa, synthetic construct
GGDGNDYMH

SEQ ID NO: 10724 - protein, 9 aa, synthetic construct
GGTGADRLW

SEQ ID NO: 10725 - protein, 9 aa, synthetic construct
GGSGNDFLI

SEQ ID NO: 10726 - protein, 9 aa, synthetic construct
GGFGDDKLH

SEQ ID NO: 10727 - protein, 9 aa, synthetic construct
GGAGIDSLY

SEQ ID NO: 10728 - protein, 9 aa, synthetic construct
GGSGNDSIL

SEQ ID NO: 10729 - protein, 9 aa, synthetic construct
GGSGHDHLY

SEQ ID NO: 10730 - protein, 9 aa, synthetic construct
GGNGDDTIS

SEQ ID NO: 10731 - protein, 9 aa, synthetic construct
GGNGDDIIY

SEQ ID NO: 10732 - protein, 9 aa, synthetic construct
GGEGNDFLI

SEQ ID NO: 10733 - protein, 9 aa, synthetic construct
GGAGIDSLS

SEQ ID NO: 10734 - protein, 9 aa, synthetic construct
GGAGNDHLI

SEQ ID NO: 10735 - protein, 9 aa, synthetic construct
GGEGNDFLF

SEQ ID NO: 10736 - protein, 9 aa, synthetic construct
GGNGDDWLV

SEQ ID NO: 10737 - protein, 9 aa, synthetic construct
GGAGKDTLE

SEQ ID NO: 10738 - protein, 9 aa, synthetic construct
GGSGNDFLN

SEQ ID NO: 10739 - protein, 9 aa, synthetic construct
GGSGNDSIF

SEQ ID NO: 10740 - protein, 9 aa, synthetic construct
GGAGNDIMR

SEQ ID NO: 10741 - protein, 9 aa, synthetic construct
GGGGNDTVD

SEQ ID NO: 10742 - protein, 9 aa, synthetic construct
GGLGSDSLT

SEQ ID NO: 10743 - protein, 9 aa, synthetic construct
GGTGADYIE

SEQ ID NO: 10744 - protein, 9 aa, synthetic construct
GGSGSDRLS

SEQ ID NO: 10745 - protein, 9 aa, synthetic construct
GGAGNDIMV

SEQ ID NO: 10746 - protein, 9 aa, synthetic construct
GGLGSDLLS

SEQ ID NO: 10747 - protein, 9 aa, synthetic construct
GGGGNDTIH

SEQ ID NO: 10748 - protein, 9 aa, synthetic construct
GGTGADHFR

SEQ ID NO: 10749 - protein, 9 aa, synthetic construct
GGDGDDQIW

SEQ ID NO: 10750 - protein, 9 aa, synthetic construct
GGNGDDFIS

SEQ ID NO: 10751 - protein, 9 aa, synthetic construct
GGSGHDELH

SEQ ID NO: 10752 - protein, 9 aa, synthetic construct
GGAGNDHIS

SEQ ID NO: 10753 - protein, 9 aa, synthetic construct
GGFGNDLLY

SEQ ID NO: 10754 - protein, 9 aa, synthetic construct
GGAGIDSMV

SEQ ID NO: 10755 - protein, 9 aa, synthetic construct
GGKGHDLLS

SEQ ID NO: 10756 - protein, 9 aa, synthetic construct
GGKGIDTII

SEQ ID NO: 10757 - protein, 9 aa, synthetic construct
GGDGNDTAF

SEQ ID NO: 10758 - protein, 9 aa, synthetic construct
GGAGNDDLT

SEQ ID NO: 10759 - protein, 9 aa, synthetic construct
GGKGNDELY

SEQ ID NO: 10760 - protein, 9 aa, synthetic construct
GGSGSDTFD

SEQ ID NO: 10761 - protein, 9 aa, synthetic construct
GGLGSDNLT

SEQ ID NO: 10762 - protein, 9 aa, synthetic construct
GGLGSDRLE

SEQ ID NO: 10763 - protein, 9 aa, synthetic construct
GGSGQDTIS

SEQ ID NO: 10764 - protein, 9 aa, synthetic construct
GGTGADELW

SEQ ID NO: 10765 - protein, 9 aa, synthetic construct
GGSGNDEIY

SEQ ID NO: 10766 - protein, 9 aa, synthetic construct
GGFGDDTIA

SEQ ID NO: 10767 - protein, 9 aa, synthetic construct
GGSGRDVLN

SEQ ID NO: 10768 - protein, 9 aa, synthetic construct
GGIGVDTLI

SEQ ID NO: 10769 - protein, 9 aa, synthetic construct
GGKGHDSIV

SEQ ID NO: 10770 - protein, 9 aa, synthetic construct
GGIGVDTLT

SEQ ID NO: 10771 - protein, 9 aa, synthetic construct
GGSGSDTAR

SEQ ID NO: 10772 - protein, 9 aa, synthetic construct
GGSGNDELL

SEQ ID NO: 10773 - protein, 9 aa, synthetic construct
GGDGNDWLN

SEQ ID NO: 10774 - protein, 9 aa, synthetic construct
GGAGKDILN

SEQ ID NO: 10775 - protein, 9 aa, synthetic construct
GGSGRDVLL

SEQ ID NO: 10776 - protein, 9 aa, synthetic construct
GGSGQDTLD

SEQ ID NO: 10777 - protein, 9 aa, synthetic construct
GGEGMDTAV

SEQ ID NO: 10778 - protein, 9 aa, synthetic construct
GGSGSDYIS

SEQ ID NO: 10779 - protein, 9 aa, synthetic construct
GGAGIDMLD

SEQ ID NO: 10780 - protein, 9 aa, synthetic construct
GGDGQDTLD

SEQ ID NO: 10781 - protein, 9 aa, synthetic construct
GGAGKDTIT

SEQ ID NO: 10782 - protein, 9 aa, synthetic construct
GGTGADRVF

SEQ ID NO: 10783 - protein, 9 aa, synthetic construct
GGSGSDEIH

SEQ ID NO: 10784 - protein, 9 aa, synthetic construct
GGSGNDSIW

SEQ ID NO: 10785 - protein, 9 aa, synthetic construct
GGDGNDRIA

SEQ ID NO: 10786 - protein, 9 aa, synthetic construct
GGEGDDTIH

SEQ ID NO: 10787 - protein, 9 aa, synthetic construct
GGKGNDFLE

SEQ ID NO: 10788 - protein, 9 aa, synthetic construct
GGSGNDTMV

SEQ ID NO: 10789 - protein, 9 aa, synthetic construct
GGSGNDQLW

SEQ ID NO: 10790 - protein, 9 aa, synthetic construct
GGTGADAMT

SEQ ID NO: 10791 - protein, 9 aa, synthetic construct
GGAGKDVIG

SEQ ID NO: 10792 - protein, 9 aa, synthetic construct
GGNGDDTIF

SEQ ID NO: 10793 - protein, 9 aa, synthetic construct
GGSGNDYVD

SEQ ID NO: 10794 - protein, 9 aa, synthetic construct
GGAGHDSLR

SEQ ID NO: 10795 - protein, 9 aa, synthetic construct
GGSGGDQLF

SEQ ID NO: 10796 - protein, 9 aa, synthetic construct
GGKGADLLI

SEQ ID NO: 10797 - protein, 9 aa, synthetic construct
GGTGADLIE

SEQ ID NO: 10798 - protein, 9 aa, synthetic construct
GGFGNDILI

SEQ ID NO: 10799 - protein, 9 aa, synthetic construct
GGSGNDLMF

SEQ ID NO: 10800 - protein, 9 aa, synthetic construct
GGSGGDLLD

SEQ ID NO: 10801 - protein, 9 aa, synthetic construct
GGKGADLLD

SEQ ID NO: 10802 - protein, 9 aa, synthetic construct
GGAGLDSID

SEQ ID NO: 10803 - protein, 9 aa, synthetic construct
GGAGIDILN

SEQ ID NO: 10804 - protein, 9 aa, synthetic construct
GGSGTDTID

SEQ ID NO: 10805 - protein, 9 aa, synthetic construct
GGGGHDVLI

SEQ ID NO: 10806 - protein, 9 aa, synthetic construct
GGAGLDTFK

SEQ ID NO: 10807 - protein, 9 aa, synthetic construct
GGNGDDHLL

SEQ ID NO: 10808 - protein, 9 aa, synthetic construct
GGSGNDLIN

SEQ ID NO: 10809 - protein, 9 aa, synthetic construct
GGKGDDTLS

SEQ ID NO: 10810 - protein, 9 aa, synthetic construct
GGTGADLIF

SEQ ID NO: 10811 - protein, 9 aa, synthetic construct
GGSGNDMLL

SEQ ID NO: 10812 - protein, 9 aa, synthetic construct
GGEGKDTFV

SEQ ID NO: 10813 - protein, 9 aa, synthetic construct
GGKGNDKLI

SEQ ID NO: 10814 - protein, 9 aa, synthetic construct
GGKGNDIYV

SEQ ID NO: 10815 - protein, 9 aa, synthetic construct
GGDGNDYIN

SEQ ID NO: 10816 - protein, 9 aa, synthetic construct
GGSGRDLLS

SEQ ID NO: 10817 - protein, 9 aa, synthetic construct
GGFGDDRLD

SEQ ID NO: 10818 - protein, 9 aa, synthetic construct
GGTGDDFLV

SEQ ID NO: 10819 - protein, 9 aa, synthetic construct
GGSGNDLFI

SEQ ID NO: 10820 - protein, 9 aa, synthetic construct
GGKGADKLT

SEQ ID NO: 10821 - protein, 9 aa, synthetic construct
GGAGNDFIA

SEQ ID NO: 10822 - protein, 9 aa, synthetic construct
GGNGDDVLQ

SEQ ID NO: 10823 - protein, 9 aa, synthetic construct
GGDGNDSIA

SEQ ID NO: 10824 - protein, 9 aa, synthetic construct
GGNGDDVLT

SEQ ID NO: 10825 - protein, 9 aa, synthetic construct
GGSGKDLLS

SEQ ID NO: 10826 - protein, 9 aa, synthetic construct
GGAGIDVLA

SEQ ID NO: 10827 - protein, 9 aa, synthetic construct
GGSGRDLFV

SEQ ID NO: 10828 - protein, 9 aa, synthetic construct
GGGGGDLLD

SEQ ID NO: 10829 - protein, 9 aa, synthetic construct
GGAGHDSLY

SEQ ID NO: 10830 - protein, 9 aa, synthetic construct
GGTGADLMD

SEQ ID NO: 10831 - protein, 9 aa, synthetic construct
GGKGDDTYY

SEQ ID NO: 10832 - protein, 9 aa, synthetic construct
GGAGKDWLE

SEQ ID NO: 10833 - protein, 9 aa, synthetic construct
GGAGNDFIY

SEQ ID NO: 10834 - protein, 9 aa, synthetic construct
GGSGVDELR

SEQ ID NO: 10835 - protein, 9 aa, synthetic construct
GGKGADVLT

SEQ ID NO: 10836 - protein, 9 aa, synthetic construct
GGSGNDWVY

SEQ ID NO: 10837 - protein, 9 aa, synthetic construct
GGEGADVLT

SEQ ID NO: 10838 - protein, 9 aa, synthetic construct
GGKGDDLII

SEQ ID NO: 10839 - protein, 9 aa, synthetic construct
GGAGKDALY

SEQ ID NO: 10840 - protein, 9 aa, synthetic construct
GGDGNDSIH

SEQ ID NO: 10841 - protein, 9 aa, synthetic construct
GGSGNDNIG

SEQ ID NO: 10842 - protein, 9 aa, synthetic construct
GGTGADLVF

SEQ ID NO: 10843 - protein, 9 aa, synthetic construct
GGDGNDVVN

SEQ ID NO: 10844 - protein, 9 aa, synthetic construct
GGIGSDTLN

SEQ ID NO: 10845 - protein, 9 aa, synthetic construct
GGAGKDVFR

SEQ ID NO: 10846 - protein, 9 aa, synthetic construct
GGDGDDMLL

SEQ ID NO: 10847 - protein, 9 aa, synthetic construct
GGSGGDRFV

SEQ ID NO: 10848 - protein, 9 aa, synthetic construct
GGAGNDKLW

SEQ ID NO: 10849 - protein, 9 aa, synthetic construct
GGAGNDLAD

SEQ ID NO: 10850 - protein, 9 aa, synthetic construct
GGDGQDSLF

SEQ ID NO: 10851 - protein, 9 aa, synthetic construct
GGAGMDNVT

SEQ ID NO: 10852 - protein, 9 aa, synthetic construct
GGGGNDSLI

SEQ ID NO: 10853 - protein, 9 aa, synthetic construct
GGAGIDWLD

SEQ ID NO: 10854 - protein, 9 aa, synthetic construct
GGDGNDTMA

SEQ ID NO: 10855 - protein, 9 aa, synthetic construct
GGEGNDELS

SEQ ID NO: 10856 - protein, 9 aa, synthetic construct
GGSGNDNIT

SEQ ID NO: 10857 - protein, 9 aa, synthetic construct
GGEGNDIFR

SEQ ID NO: 10858 - protein, 9 aa, synthetic construct
GGKGNDKLF

SEQ ID NO: 10859 - protein, 9 aa, synthetic construct
GGFGNDIIN

SEQ ID NO: 10860 - protein, 9 aa, synthetic construct
GGSGNDLYI

SEQ ID NO: 10861 - protein, 9 aa, synthetic construct
GGSGRDQLT

SEQ ID NO: 10862 - protein, 9 aa, synthetic construct
GGSGRDRLF

SEQ ID NO: 10863 - protein, 9 aa, synthetic construct
GGAGHDSLL

SEQ ID NO: 10864 - protein, 9 aa, synthetic construct
GGSGNDQLT

SEQ ID NO: 10865 - protein, 9 aa, synthetic construct
GGTGADNLI

SEQ ID NO: 10866 - protein, 9 aa, synthetic construct
GGSGNDYIE

SEQ ID NO: 10867 - protein, 9 aa, synthetic construct
GGSGVDIFV

SEQ ID NO: 10868 - protein, 9 aa, synthetic construct
GGSGNDLVY

SEQ ID NO: 10869 - protein, 9 aa, synthetic construct
GGLGSDTFI

SEQ ID NO: 10870 - protein, 9 aa, synthetic construct
GGAGLDSLI

SEQ ID NO: 10871 - protein, 9 aa, synthetic construct
GGDGQDSLI

SEQ ID NO: 10872 - protein, 9 aa, synthetic construct
GGDGNDRVY

SEQ ID NO: 10873 - protein, 9 aa, synthetic construct
GGTGRDRLN

SEQ ID NO: 10874 - protein, 9 aa, synthetic construct
GGTGNDQMT

SEQ ID NO: 10875 - protein, 9 aa, synthetic construct
GGDGDDTIM

SEQ ID NO: 10876 - protein, 9 aa, synthetic construct
GGDGDDSVG

SEQ ID NO: 10877 - protein, 9 aa, synthetic construct
GGEGRDTLS

SEQ ID NO: 10878 - protein, 9 aa, synthetic construct
GGMGHDTLN

SEQ ID NO: 10879 - protein, 9 aa, synthetic construct
GGTGRDRFV

SEQ ID NO: 10880 - protein, 9 aa, synthetic construct
GGAGRDKLD

SEQ ID NO: 10881 - protein, 9 aa, synthetic construct
GGLGKDVID

SEQ ID NO: 10882 - protein, 9 aa, synthetic construct
GGEGADVLR

SEQ ID NO: 10883 - protein, 9 aa, synthetic construct
GGPGNDQLS

SEQ ID NO: 10884 - protein, 9 aa, synthetic construct
GGEGDDALN

SEQ ID NO: 10885 - protein, 9 aa, synthetic construct
GGEGRDTLR

SEQ ID NO: 10886 - protein, 9 aa, synthetic construct
GGLGADALI

SEQ ID NO: 10887 - protein, 9 aa, synthetic construct
GGAGKDKMF

SEQ ID NO: 10888 - protein, 9 aa, synthetic construct
GGDGNDHLN

SEQ ID NO: 10889 - protein, 9 aa, synthetic construct
GGIGDDELD

SEQ ID NO: 10890 - protein, 9 aa, synthetic construct
GGVGSDYLG

SEQ ID NO: 10891 - protein, 9 aa, synthetic construct
GGAGEDAIF

SEQ ID NO: 10892 - protein, 9 aa, synthetic construct
GGDGNDVFL

SEQ ID NO: 10893 - protein, 9 aa, synthetic construct
GGDGSDSLI

SEQ ID NO: 10894 - protein, 9 aa, synthetic construct
GGTGRDSMA

SEQ ID NO: 10895 - protein, 9 aa, synthetic construct
GGRGDDYLD

SEQ ID NO: 10896 - protein, 9 aa, synthetic construct
GGDGHDTAL

SEQ ID NO: 10897 - protein, 9 aa, synthetic construct
GGWGNDSLA

SEQ ID NO: 10898 - protein, 9 aa, synthetic construct
GGGGDDLLQ

SEQ ID NO: 10899 - protein, 9 aa, synthetic construct
GGAGADVYV

SEQ ID NO: 10900 - protein, 9 aa, synthetic construct
GGTGADLMQ

SEQ ID NO: 10901 - protein, 9 aa, synthetic construct
GGGGRDVFV

SEQ ID NO: 10902 - protein, 9 aa, synthetic construct
GGAGQDEVT

SEQ ID NO: 10903 - protein, 9 aa, synthetic construct
GGLGKDTVS

SEQ ID NO: 10904 - protein, 9 aa, synthetic construct
GGLGRDVLL

SEQ ID NO: 10905 - protein, 9 aa, synthetic construct
GGPGDDRLA

SEQ ID NO: 10906 - protein, 9 aa, synthetic construct
GGSGKDIMT

SEQ ID NO: 10907 - protein, 9 aa, synthetic construct
GGTGRDTIN

SEQ ID NO: 10908 - protein, 9 aa, synthetic construct
GGLGADVIY

SEQ ID NO: 10909 - protein, 9 aa, synthetic construct
GGGGADAMF

SEQ ID NO: 10910 - protein, 9 aa, synthetic construct
GGSGSDTFA

SEQ ID NO: 10911 - protein, 9 aa, synthetic construct
GGAGRDLID

SEQ ID NO: 10912 - protein, 9 aa, synthetic construct
GGAGVDKLY

SEQ ID NO: 10913 - protein, 9 aa, synthetic construct
GGAGADRII

SEQ ID NO: 10914 - protein, 9 aa, synthetic construct
GGIGDDALY

SEQ ID NO: 10915 - protein, 9 aa, synthetic construct
GGLGQDRLD

SEQ ID NO: 10916 - protein, 9 aa, synthetic construct
GGVGSDVLD

SEQ ID NO: 10917 - protein, 9 aa, synthetic construct
GGDGNDEAF

SEQ ID NO: 10918 - protein, 9 aa, synthetic construct
GGTGRDSLD

SEQ ID NO: 10919 - protein, 9 aa, synthetic construct
GGVGSDVLE

SEQ ID NO: 10920 - protein, 9 aa, synthetic construct
GGGGNDIMS

SEQ ID NO: 10921 - protein, 9 aa, synthetic construct
GGLGADVID

SEQ ID NO: 10922 - protein, 9 aa, synthetic construct
GGVGSDVLF

SEQ ID NO: 10923 - protein, 9 aa, synthetic construct
GGVGSDVLN

SEQ ID NO: 10924 - protein, 9 aa, synthetic construct
GGPGNDRLN

SEQ ID NO: 10925 - protein, 9 aa, synthetic construct
GGEGMDHLS

SEQ ID NO: 10926 - protein, 9 aa, synthetic construct
GGSGLDSID

SEQ ID NO: 10927 - protein, 9 aa, synthetic construct
GGSGSDSLY

SEQ ID NO: 10928 - protein, 9 aa, synthetic construct
GGAGEDILA

SEQ ID NO: 10929 - protein, 9 aa, synthetic construct
GGTGADFLT

SEQ ID NO: 10930 - protein, 9 aa, synthetic construct
GGTGRDIFV

SEQ ID NO: 10931 - protein, 9 aa, synthetic construct
GGGGKDTLL

SEQ ID NO: 10932 - protein, 9 aa, synthetic construct
GGAGADRIR

SEQ ID NO: 10933 - protein, 9 aa, synthetic construct
GGGGDDLYY

SEQ ID NO: 10934 - protein, 9 aa, synthetic construct
GGSGSDSIF

SEQ ID NO: 10935 - protein, 9 aa, synthetic construct
GGAGRDHVS

SEQ ID NO: 10936 - protein, 9 aa, synthetic construct
GGLGNDIFI

SEQ ID NO: 10937 - protein, 9 aa, synthetic construct
GGLGADTLH

SEQ ID NO: 10938 - protein, 9 aa, synthetic construct
GGSGKDKLD

SEQ ID NO: 10939 - protein, 9 aa, synthetic construct
GGDGNDHLH

SEQ ID NO: 10940 - protein, 9 aa, synthetic construct
GGLGLDLLY

SEQ ID NO: 10941 - protein, 9 aa, synthetic construct
GGRGGDTLL

SEQ ID NO: 10942 - protein, 9 aa, synthetic construct
GGDGDDYVD

SEQ ID NO: 10943 - protein, 9 aa, synthetic construct
GGLGNDIFL

SEQ ID NO: 10944 - protein, 9 aa, synthetic construct
GGDGFDLLN

SEQ ID NO: 10945 - protein, 9 aa, synthetic construct
GGFGNDTVL

SEQ ID NO: 10946 - protein, 9 aa, synthetic construct
GGIGDDIIM

SEQ ID NO: 10947 - protein, 9 aa, synthetic construct
GGIGDDIII

SEQ ID NO: 10948 - protein, 9 aa, synthetic construct
GGRGRDLID

SEQ ID NO: 10949 - protein, 9 aa, synthetic construct
GGRGGDTID

SEQ ID NO: 10950 - protein, 9 aa, synthetic construct
GGLGADTIT

SEQ ID NO: 10951 - protein, 9 aa, synthetic construct
GGDGVDVLF

SEQ ID NO: 10952 - protein, 9 aa, synthetic construct
GGSGSDSLR

SEQ ID NO: 10953 - protein, 9 aa, synthetic construct
GGPGNDILT

SEQ ID NO: 10954 - protein, 9 aa, synthetic construct
GGAGADVLG

SEQ ID NO: 10955 - protein, 9 aa, synthetic construct
GGAGKDLIL

SEQ ID NO: 10956 - protein, 9 aa, synthetic construct
GGAGIDLLY

SEQ ID NO: 10957 - protein, 9 aa, synthetic construct
GGAGIDLME

SEQ ID NO: 10958 - protein, 9 aa, synthetic construct
GGDGNDYME

SEQ ID NO: 10959 - protein, 9 aa, synthetic construct
GGTGADFLV

SEQ ID NO: 10960 - protein, 9 aa, synthetic construct
GGAGEDILN

SEQ ID NO: 10961 - protein, 9 aa, synthetic construct
GGKGIDTMI

SEQ ID NO: 10962 - protein, 9 aa, synthetic construct
GGWGNDQLF

SEQ ID NO: 10963 - protein, 9 aa, synthetic construct
GGGGADDIG

SEQ ID NO: 10964 - protein, 9 aa, synthetic construct
GGLGADTIE

SEQ ID NO: 10965 - protein, 9 aa, synthetic construct
GGDGNDHLD

SEQ ID NO: 10966 - protein, 9 aa, synthetic construct
GGFGNDTYH

SEQ ID NO: 10967 - protein, 9 aa, synthetic construct
GGNGDDTIL

SEQ ID NO: 10968 - protein, 9 aa, synthetic construct
GGAGRDHLF

SEQ ID NO: 10969 - protein, 9 aa, synthetic construct
GGSGLDNLD

SEQ ID NO: 10970 - protein, 9 aa, synthetic construct
GGLGNDIFE

SEQ ID NO: 10971 - protein, 9 aa, synthetic construct
GGAGVDNIN

SEQ ID NO: 10972 - protein, 9 aa, synthetic construct
GGVGTDTLD

SEQ ID NO: 10973 - protein, 9 aa, synthetic construct
GGPGNDILS

SEQ ID NO: 10974 - protein, 9 aa, synthetic construct
GGAGRDHLR

SEQ ID NO: 10975 - protein, 9 aa, synthetic construct
GGDGQDNLY

SEQ ID NO: 10976 - protein, 9 aa, synthetic construct
GGIGDDVLA

SEQ ID NO: 10977 - protein, 9 aa, synthetic construct
GGTGRDLAD

SEQ ID NO: 10978 - protein, 9 aa, synthetic construct
GGTGRDLAH

SEQ ID NO: 10979 - protein, 9 aa, synthetic construct
GGTGRDLYL

SEQ ID NO: 10980 - protein, 9 aa, synthetic construct
GGWGNDRLH

SEQ ID NO: 10981 - protein, 9 aa, synthetic construct
GGSGSDSLL

SEQ ID NO: 10982 - protein, 9 aa, synthetic construct
GGAGVDLMR

SEQ ID NO: 10983 - protein, 9 aa, synthetic construct
GGAGRDIMT

SEQ ID NO: 10984 - protein, 9 aa, synthetic construct
GGDGIDLAD

SEQ ID NO: 10985 - protein, 9 aa, synthetic construct
GGRGRDLMF

SEQ ID NO: 10986 - protein, 9 aa, synthetic construct
GGVGSDTLY

SEQ ID NO: 10987 - protein, 9 aa, synthetic construct
GGPGNDLYL

SEQ ID NO: 10988 - protein, 9 aa, synthetic construct
GGLGADALY

SEQ ID NO: 10989 - protein, 9 aa, synthetic construct
GGHGADELH

SEQ ID NO: 10990 - protein, 9 aa, synthetic construct
GGGGIDTLF

SEQ ID NO: 10991 - protein, 9 aa, synthetic construct
GGAGEDYLY

SEQ ID NO: 10992 - protein, 9 aa, synthetic construct
GGDGDDLVT

SEQ ID NO: 10993 - protein, 9 aa, synthetic construct
GGAGRDIVV

SEQ ID NO: 10994 - protein, 9 aa, synthetic construct
GGLGADTVT

SEQ ID NO: 10995 - protein, 9 aa, synthetic construct
GGAGEDDLR

SEQ ID NO: 10996 - protein, 9 aa, synthetic construct
GGFGNDTMY

SEQ ID NO: 10997 - protein, 9 aa, synthetic construct
GGTGRDQIG

SEQ ID NO: 10998 - protein, 9 aa, synthetic construct
GGEGRDTLM

SEQ ID NO: 10999 - protein, 9 aa, synthetic construct
GGSGLDSLY

SEQ ID NO: 11000 - protein, 9 aa, synthetic construct
GGDGIDKAV

SEQ ID NO: 11001 - protein, 9 aa, synthetic construct
GGKGIDTAS

SEQ ID NO: 11002 - protein, 9 aa, synthetic construct
GGAGIDMAS

SEQ ID NO: 11003 - protein, 9 aa, synthetic construct
GGGGFDTVS

SEQ ID NO: 11004 - protein, 9 aa, synthetic construct
GGRGRDLLD

SEQ ID NO: 11005 - protein, 9 aa, synthetic construct
GGAGRDIIH

SEQ ID NO: 11006 - protein, 9 aa, synthetic construct
GGAGQDHYR

SEQ ID NO: 11007 - protein, 9 aa, synthetic construct
GGLGADAMQ

SEQ ID NO: 11008 - protein, 9 aa, synthetic construct
GGTGRDLLD

SEQ ID NO: 11009 - protein, 9 aa, synthetic construct
GGDGDDSVL

SEQ ID NO: 11010 - protein, 9 aa, synthetic construct
GGAGRDIIV

SEQ ID NO: 11011 - protein, 9 aa, synthetic construct
GGEGADLIY

SEQ ID NO: 11012 - protein, 9 aa, synthetic construct
GGNGHDTFV

SEQ ID NO: 11013 - protein, 9 aa, synthetic construct
GGSGNDTMY

SEQ ID NO: 11014 - protein, 9 aa, synthetic construct
GGDGSDLIS

SEQ ID NO: 11015 - protein, 9 aa, synthetic construct
GGDGNDEIH

SEQ ID NO: 11016 - protein, 9 aa, synthetic construct
GGDGSDRLM

SEQ ID NO: 11017 - protein, 9 aa, synthetic construct
GGDGSDRLN

SEQ ID NO: 11018 - protein, 9 aa, synthetic construct
GGSGLDRFY

SEQ ID NO: 11019 - protein, 9 aa, synthetic construct
GGDGDDHII

SEQ ID NO: 11020 - protein, 9 aa, synthetic construct
GGAGEDELR

SEQ ID NO: 11021 - protein, 9 aa, synthetic construct
GGSGLDRLF

SEQ ID NO: 11022 - protein, 9 aa, synthetic construct
GGVGTDLLT

SEQ ID NO: 11023 - protein, 9 aa, synthetic construct
GGSGSDSIW

SEQ ID NO: 11024 - protein, 9 aa, synthetic construct
GGTGADELT

SEQ ID NO: 11025 - protein, 9 aa, synthetic construct
GGEGTDTLI

SEQ ID NO: 11026 - protein, 9 aa, synthetic construct
GGDGSDSLS

SEQ ID NO: 11027 - protein, 9 aa, synthetic construct
GGSGSDTLW

SEQ ID NO: 11028 - protein, 9 aa, synthetic construct
GGNGADAVI

SEQ ID NO: 11029 - protein, 9 aa, synthetic construct
GGTGSDIYD

SEQ ID NO: 11030 - protein, 9 aa, synthetic construct
GGDGDDHLS

SEQ ID NO: 11031 - protein, 9 aa, synthetic construct
GGIGADTLK

SEQ ID NO: 11032 - protein, 9 aa, synthetic construct
GGAGRDQIT

SEQ ID NO: 11033 - protein, 9 aa, synthetic construct
GGPGNDVLN

SEQ ID NO: 11034 - protein, 9 aa, synthetic construct
GGIGADTLF

SEQ ID NO: 11035 - protein, 9 aa, synthetic construct
GGVGSDKLY

SEQ ID NO: 11036 - protein, 9 aa, synthetic construct
GGDGNDSVR

SEQ ID NO: 11037 - protein, 9 aa, synthetic construct
GGRGRDYLS

SEQ ID NO: 11038 - protein, 9 aa, synthetic construct
GGDGEDIIK

SEQ ID NO: 11039 - protein, 9 aa, synthetic construct
GGTGNDNLF

SEQ ID NO: 11040 - protein, 9 aa, synthetic construct
GGEGRDVLF

SEQ ID NO: 11041 - protein, 9 aa, synthetic construct
GGRGDDMLD

SEQ ID NO: 11042 - protein, 9 aa, synthetic construct
GGPGDDLLQ

SEQ ID NO: 11043 - protein, 9 aa, synthetic construct
GGAGADQMN

SEQ ID NO: 11044 - protein, 9 aa, synthetic construct
GGAGRDQLS

SEQ ID NO: 11045 - protein, 9 aa, synthetic construct
GGMGDDTYV

SEQ ID NO: 11046 - protein, 9 aa, synthetic construct
GGAGFDFAD

SEQ ID NO: 11047 - protein, 9 aa, synthetic construct
GGEGSDVFI

SEQ ID NO: 11048 - protein, 9 aa, synthetic construct
GGNGHDVYQ

SEQ ID NO: 11049 - protein, 9 aa, synthetic construct
GGDGEDIIF

SEQ ID NO: 11050 - protein, 9 aa, synthetic construct
GGRGDDQLD

SEQ ID NO: 11051 - protein, 9 aa, synthetic construct
GGEGVDFLE

SEQ ID NO: 11052 - protein, 9 aa, synthetic construct
GGVGSDQLH

SEQ ID NO: 11053 - protein, 9 aa, synthetic construct
GGGGADMFV

SEQ ID NO: 11054 - protein, 9 aa, synthetic construct
GGLGRDVLV

SEQ ID NO: 11055 - protein, 9 aa, synthetic construct
GGTGSDHLL

SEQ ID NO: 11056 - protein, 9 aa, synthetic construct
GGRGDDRLA

SEQ ID NO: 11057 - protein, 9 aa, synthetic construct
GGPGNDTYI

SEQ ID NO: 11058 - protein, 9 aa, synthetic construct
GGDGNDDLF

SEQ ID NO: 11059 - protein, 9 aa, synthetic construct
GGKGADTFE

SEQ ID NO: 11060 - protein, 9 aa, synthetic construct
GGPGNDVID

SEQ ID NO: 11061 - protein, 9 aa, synthetic construct
GGNGHDVLN

SEQ ID NO: 11062 - protein, 9 aa, synthetic construct
GGEGADLLR

SEQ ID NO: 11063 - protein, 9 aa, synthetic construct
GGDGNDDIS

SEQ ID NO: 11064 - protein, 9 aa, synthetic construct
GGSGSDTMV

SEQ ID NO: 11065 - protein, 9 aa, synthetic construct
GGSGSDTVA

SEQ ID NO: 11066 - protein, 9 aa, synthetic construct
GGGGRDTLY

SEQ ID NO: 11067 - protein, 9 aa, synthetic construct
GGLGADYLY

SEQ ID NO: 11068 - protein, 9 aa, synthetic construct
GGTGSDILS

SEQ ID NO: 11069 - protein, 9 aa, synthetic construct
GGDGNDIFD

SEQ ID NO: 11070 - protein, 9 aa, synthetic construct
GGRGDDQLN

SEQ ID NO: 11071 - protein, 9 aa, synthetic construct
GGTGSDIMD

SEQ ID NO: 11072 - protein, 9 aa, synthetic construct
GGAGDDWIE

SEQ ID NO: 11073 - protein, 9 aa, synthetic construct
GGIGADTIT

SEQ ID NO: 11074 - protein, 9 aa, synthetic construct
GGKGVDTVI

SEQ ID NO: 11075 - protein, 9 aa, synthetic construct
GGDGSDLFH

SEQ ID NO: 11076 - protein, 9 aa, synthetic construct
GGPGDDLIE

SEQ ID NO: 11077 - protein, 9 aa, synthetic construct
GGGGADNLF

SEQ ID NO: 11078 - protein, 9 aa, synthetic construct
GGTGNDNIF

SEQ ID NO: 11079 - protein, 9 aa, synthetic construct
GGKGVDTLI

SEQ ID NO: 11080 - protein, 9 aa, synthetic construct
GGAGLDSII

SEQ ID NO: 11081 - protein, 9 aa, synthetic construct
GGDGNDYVL

SEQ ID NO: 11082 - protein, 9 aa, synthetic construct
GGRGSDFLE

SEQ ID NO: 11083 - protein, 9 aa, synthetic construct
GGAGADYLL

SEQ ID NO: 11084 - protein, 9 aa, synthetic construct
GGAGPDTMI

SEQ ID NO: 11085 - protein, 9 aa, synthetic construct
GGLGDDDIG

SEQ ID NO: 11086 - protein, 9 aa, synthetic construct
GGPGDDLID

SEQ ID NO: 11087 - protein, 9 aa, synthetic construct
GGAGADQMF

SEQ ID NO: 11088 - protein, 9 aa, synthetic construct
GGKGADSLY

SEQ ID NO: 11089 - protein, 9 aa, synthetic construct
GGDGIDRLD

SEQ ID NO: 11090 - protein, 9 aa, synthetic construct
GGRGDDIYI

SEQ ID NO: 11091 - protein, 9 aa, synthetic construct
GGLGKDMLI

SEQ ID NO: 11092 - protein, 9 aa, synthetic construct
GGAGADYLY

SEQ ID NO: 11093 - protein, 9 aa, synthetic construct
GGVGSDALN

SEQ ID NO: 11094 - protein, 9 aa, synthetic construct
GGDGVDYLT

SEQ ID NO: 11095 - protein, 9 aa, synthetic construct
GGLGKDLLT

SEQ ID NO: 11096 - protein, 9 aa, synthetic construct
GGTGSDNLR

SEQ ID NO: 11097 - protein, 9 aa, synthetic construct
GGAGIDQLF

SEQ ID NO: 11098 - protein, 9 aa, synthetic construct
GGRGDDLIA

SEQ ID NO: 11099 - protein, 9 aa, synthetic construct
GGEGEDVFV

SEQ ID NO: 11100 - protein, 9 aa, synthetic construct
GGTGSDLLY

SEQ ID NO: 11101 - protein, 9 aa, synthetic construct
GGFGNDTLK

SEQ ID NO: 11102 - protein, 9 aa, synthetic construct
GGLGDDALT

SEQ ID NO: 11103 - protein, 9 aa, synthetic construct
GGGGNDILC

SEQ ID NO: 11104 - protein, 9 aa, synthetic construct
GGAGRDRAQ

SEQ ID NO: 11105 - protein, 9 aa, synthetic construct
GGDGDDFAS

SEQ ID NO: 11106 - protein, 9 aa, synthetic construct
GGIGADTIL

SEQ ID NO: 11107 - protein, 9 aa, synthetic construct
GGDGIDQLY

SEQ ID NO: 11108 - protein, 9 aa, synthetic construct
GGSGNDTFF

SEQ ID NO: 11109 - protein, 9 aa, synthetic construct
GGRGDDLLN

SEQ ID NO: 11110 - protein, 9 aa, synthetic construct
GGGGNDILA

SEQ ID NO: 11111 - protein, 9 aa, synthetic construct
GGAGNDAYV

SEQ ID NO: 11112 - protein, 9 aa, synthetic construct
GGAGRDRFL

SEQ ID NO: 11113 - protein, 9 aa, synthetic construct
GGAGDDVVN

SEQ ID NO: 11114 - protein, 9 aa, synthetic construct
GGGGNDIIY

SEQ ID NO: 11115 - protein, 9 aa, synthetic construct
GGAGADYIE

SEQ ID NO: 11116 - protein, 9 aa, synthetic construct
GGKGVDTMI

SEQ ID NO: 11117 - protein, 9 aa, synthetic construct
GGDGDDYIV

SEQ ID NO: 11118 - protein, 9 aa, synthetic construct
GGAGYDLIV

SEQ ID NO: 11119 - protein, 9 aa, synthetic construct
GGDGEDILD

SEQ ID NO: 11120 - protein, 9 aa, synthetic construct
GGSGSDTVS

SEQ ID NO: 11121 - protein, 9 aa, synthetic construct
GGRGDDRLI

SEQ ID NO: 11122 - protein, 9 aa, synthetic construct
GGRGRDVMN

SEQ ID NO: 11123 - protein, 9 aa, synthetic construct
GGSGSDTFI

SEQ ID NO: 11124 - protein, 9 aa, synthetic construct
GGIGSDTYI

SEQ ID NO: 11125 - protein, 9 aa, synthetic construct
GGPGNDSMG

SEQ ID NO: 11126 - protein, 9 aa, synthetic construct
GGLGADVMD

SEQ ID NO: 11127 - protein, 9 aa, synthetic construct
GGAGDDYIS

SEQ ID NO: 11128 - protein, 9 aa, synthetic construct
GGLGRDVLN

SEQ ID NO: 11129 - protein, 9 aa, synthetic construct
GGEGGDVLR

SEQ ID NO: 11130 - protein, 9 aa, synthetic construct
GGSGKDILI

SEQ ID NO: 11131 - protein, 9 aa, synthetic construct
GGTGADEIF

SEQ ID NO: 11132 - protein, 9 aa, synthetic construct
GGAGNDFIS

SEQ ID NO: 11133 - protein, 9 aa, synthetic construct
GGAGADWID

SEQ ID NO: 11134 - protein, 9 aa, synthetic construct
GGRGDDTLY

SEQ ID NO: 11135 - protein, 9 aa, synthetic construct
GGTGNDQID

SEQ ID NO: 11136 - protein, 9 aa, synthetic construct
GGPGDDQLF

SEQ ID NO: 11137 - protein, 9 aa, synthetic construct
GGDGNDVFN

SEQ ID NO: 11138 - protein, 9 aa, synthetic construct
GGTGADEID

SEQ ID NO: 11139 - protein, 9 aa, synthetic construct
GGIGTDVAR

SEQ ID NO: 11140 - protein, 9 aa, synthetic construct
GGDGFDLLD

SEQ ID NO: 11141 - protein, 9 aa, synthetic construct
GGRGDDTLR

SEQ ID NO: 11142 - protein, 9 aa, synthetic construct
GGVGSDTFI

SEQ ID NO: 11143 - protein, 9 aa, synthetic construct
GGRGDDTLM

SEQ ID NO: 11144 - protein, 9 aa, synthetic construct
GGTGRDYLD

SEQ ID NO: 11145 - protein, 9 aa, synthetic construct
GGAGNDDIT

SEQ ID NO: 11146 - protein, 9 aa, synthetic construct
GGDGNDSVF

SEQ ID NO: 11147 - protein, 9 aa, synthetic construct
GGAGRDLLV

SEQ ID NO: 11148 - protein, 9 aa, synthetic construct
GGAGADRFS

SEQ ID NO: 11149 - protein, 9 aa, synthetic construct
GGAGNDDLG

SEQ ID NO: 11150 - protein, 9 aa, synthetic construct
GGVGSDTLT

SEQ ID NO: 11151 - protein, 9 aa, synthetic construct
GGAGVDKLF

SEQ ID NO: 11152 - protein, 9 aa, synthetic construct
GGIGTDTLN

SEQ ID NO: 11153 - protein, 9 aa, synthetic construct
GGSGLDTVV

SEQ ID NO: 11154 - protein, 9 aa, synthetic construct
GGGGIDTLA

SEQ ID NO: 11155 - protein, 9 aa, synthetic construct
GGTGADEIT

SEQ ID NO: 11156 - protein, 9 aa, synthetic construct
GGTGRDTMT

SEQ ID NO: 11157 - protein, 9 aa, synthetic construct
GGTGRDVID

SEQ ID NO: 11158 - protein, 9 aa, synthetic construct
GGGGDDSIY

SEQ ID NO: 11159 - protein, 9 aa, synthetic construct
GGIGADVMS

SEQ ID NO: 11160 - protein, 9 aa, synthetic construct
GGPGNDSLY

SEQ ID NO: 11161 - protein, 9 aa, synthetic construct
GGAGRDLLQ

SEQ ID NO: 11162 - protein, 9 aa, synthetic construct
GGRGDDVIL

SEQ ID NO: 11163 - protein, 9 aa, synthetic construct
GGRGDDVIE

SEQ ID NO: 11164 - protein, 9 aa, synthetic construct
GGDGSDLIF

SEQ ID NO: 11165 - protein, 9 aa, synthetic construct
GGGGDDLLH

SEQ ID NO: 11166 - protein, 9 aa, synthetic construct
GGVGTDVLF

SEQ ID NO: 11167 - protein, 9 aa, synthetic construct
GGGGADALN

SEQ ID NO: 11168 - protein, 9 aa, synthetic construct
GGDGNDSVE

SEQ ID NO: 11169 - protein, 9 aa, synthetic construct
GGRGDDTYL

SEQ ID NO: 11170 - protein, 9 aa, synthetic construct
GGAGDDYIF

SEQ ID NO: 11171 - protein, 9 aa, synthetic construct
GGVGSDTAS

SEQ ID NO: 11172 - protein, 9 aa, synthetic construct
GGKGYDQIH

SEQ ID NO: 11173 - protein, 9 aa, synthetic construct
GGTGSDFLA

SEQ ID NO: 11174 - protein, 9 aa, synthetic construct
GGTGNDNMI

SEQ ID NO: 11175 - protein, 9 aa, synthetic construct
GGIGADTMN

SEQ ID NO: 11176 - protein, 9 aa, synthetic construct
GGSGNDTIM

SEQ ID NO: 11177 - protein, 9 aa, synthetic construct
GGGGDDSLQ

SEQ ID NO: 11178 - protein, 9 aa, synthetic construct
GGAGNDFIT

SEQ ID NO: 11179 - protein, 9 aa, synthetic construct
GGLGADWLD

SEQ ID NO: 11180 - protein, 9 aa, synthetic construct
GGAGNDDIA

SEQ ID NO: 11181 - protein, 9 aa, synthetic construct
GGRGRDVLI

SEQ ID NO: 11182 - protein, 9 aa, synthetic construct
GGAGVDILN

SEQ ID NO: 11183 - protein, 9 aa, synthetic construct
GGVGSDRLE

SEQ ID NO: 11184 - protein, 9 aa, synthetic construct
GGRGDDSLI

SEQ ID NO: 11185 - protein, 9 aa, synthetic construct
GGAGVDILD

SEQ ID NO: 11186 - protein, 9 aa, synthetic construct
GGAGDDWLK

SEQ ID NO: 11187 - protein, 9 aa, synthetic construct
GGRGDDRLY

SEQ ID NO: 11188 - protein, 9 aa, synthetic construct
GGNGNDILW

SEQ ID NO: 11189 - protein, 9 aa, synthetic construct
GGDGVDWLE

SEQ ID NO: 11190 - protein, 9 aa, synthetic construct
GGRGDDRLS

SEQ ID NO: 11191 - protein, 9 aa, synthetic construct
GGAGQDAID

SEQ ID NO: 11192 - protein, 9 aa, synthetic construct
GGAGNDDFI

SEQ ID NO: 11193 - protein, 9 aa, synthetic construct
GGAGADWLW

SEQ ID NO: 11194 - protein, 9 aa, synthetic construct
GGSGSDTLH

SEQ ID NO: 11195 - protein, 9 aa, synthetic construct
GGDGDDYLI

SEQ ID NO: 11196 - protein, 9 aa, synthetic construct
GGIGADVLI

SEQ ID NO: 11197 - protein, 9 aa, synthetic construct
GGDGVDVLR

SEQ ID NO: 11198 - protein, 9 aa, synthetic construct
GGSGSDTIN

SEQ ID NO: 11199 - protein, 9 aa, synthetic construct
GGAGNDDIS

SEQ ID NO: 11200 - protein, 9 aa, synthetic construct
GGNGNDIMV

SEQ ID NO: 11201 - protein, 9 aa, synthetic construct
GGDGSDTAI

SEQ ID NO: 11202 - protein, 9 aa, synthetic construct
GGGGDDSLG

SEQ ID NO: 11203 - protein, 9 aa, synthetic construct
GGEGGDVLD

SEQ ID NO: 11204 - protein, 9 aa, synthetic construct
GGNGHDTLV

SEQ ID NO: 11205 - protein, 9 aa, synthetic construct
GGEGSDVLV

SEQ ID NO: 11206 - protein, 9 aa, synthetic construct
GGIGADVID

SEQ ID NO: 11207 - protein, 9 aa, synthetic construct
GGEGNDVVY

SEQ ID NO: 11208 - protein, 9 aa, synthetic construct
GGGGRDYIT

SEQ ID NO: 11209 - protein, 9 aa, synthetic construct
GGAGRDMAI

SEQ ID NO: 11210 - protein, 9 aa, synthetic construct
GGAGIDNLI

SEQ ID NO: 11211 - protein, 9 aa, synthetic construct
GGLGADVVH

SEQ ID NO: 11212 - protein, 9 aa, synthetic construct
GGAGADWIY

SEQ ID NO: 11213 - protein, 9 aa, synthetic construct
GGFGDDTIL

SEQ ID NO: 11214 - protein, 9 aa, synthetic construct
GGDGSDTFL

SEQ ID NO: 11215 - protein, 9 aa, synthetic construct
GGEGNDVVV

SEQ ID NO: 11216 - protein, 9 aa, synthetic construct
GGTGNDNMT

SEQ ID NO: 11217 - protein, 9 aa, synthetic construct
GGRGDDSLN

SEQ ID NO: 11218 - protein, 9 aa, synthetic construct
GGTGRDELT

SEQ ID NO: 11219 - protein, 9 aa, synthetic construct
GGAGRDFLH

SEQ ID NO: 11220 - protein, 9 aa, synthetic construct
GGNGHDSLT

SEQ ID NO: 11221 - protein, 9 aa, synthetic construct
GGGGKDTIY

SEQ ID NO: 11222 - protein, 9 aa, synthetic construct
GGEGDDRIE

SEQ ID NO: 11223 - protein, 9 aa, synthetic construct
GGEGADSLF

SEQ ID NO: 11224 - protein, 9 aa, synthetic construct
GGDGNDYIW

SEQ ID NO: 11225 - protein, 9 aa, synthetic construct
GGRGNDVLY

SEQ ID NO: 11226 - protein, 9 aa, synthetic construct
GGWGDDRLD

SEQ ID NO: 11227 - protein, 9 aa, synthetic construct
GGTGNDYLQ

SEQ ID NO: 11228 - protein, 9 aa, synthetic construct
GGWGDDRIT

SEQ ID NO: 11229 - protein, 9 aa, synthetic construct
GGGGDDRIS

SEQ ID NO: 11230 - protein, 9 aa, synthetic construct
GGAGVDTLE

SEQ ID NO: 11231 - protein, 9 aa, synthetic construct
GGTGNDYLR

SEQ ID NO: 11232 - protein, 9 aa, synthetic construct
GGTGNDYMD

SEQ ID NO: 11233 - protein, 9 aa, synthetic construct
GGTGNDYMH

SEQ ID NO: 11234 - protein, 9 aa, synthetic construct
GGSGSDLAA

SEQ ID NO: 11235 - protein, 9 aa, synthetic construct
GGAGEDTAD

SEQ ID NO: 11236 - protein, 9 aa, synthetic construct
GGPGHDNLF

SEQ ID NO: 11237 - protein, 9 aa, synthetic construct
GGLGADIMR

SEQ ID NO: 11238 - protein, 9 aa, synthetic construct
GGLGADNLS

SEQ ID NO: 11239 - protein, 9 aa, synthetic construct
GGLGADNLT

SEQ ID NO: 11240 - protein, 9 aa, synthetic construct
GGKGKDIFV

SEQ ID NO: 11241 - protein, 9 aa, synthetic construct
GGEGNDWLE

SEQ ID NO: 11242 - protein, 9 aa, synthetic construct
GGGGADHLV

SEQ ID NO: 11243 - protein, 9 aa, synthetic construct
GGDGNDSIF

SEQ ID NO: 11244 - protein, 9 aa, synthetic construct
GGEGNDRMD

SEQ ID NO: 11245 - protein, 9 aa, synthetic construct
GGDGHDTLV

SEQ ID NO: 11246 - protein, 9 aa, synthetic construct
GGSGSDLLS

SEQ ID NO: 11247 - protein, 9 aa, synthetic construct
GGEGTDTAV

SEQ ID NO: 11248 - protein, 9 aa, synthetic construct
GGWGDDTLD

SEQ ID NO: 11249 - protein, 9 aa, synthetic construct
GGDGSDLLF

SEQ ID NO: 11250 - protein, 9 aa, synthetic construct
GGGGADFLA

SEQ ID NO: 11251 - protein, 9 aa, synthetic construct
GGGGADHLI

SEQ ID NO: 11252 - protein, 9 aa, synthetic construct
GGWGDDTIY

SEQ ID NO: 11253 - protein, 9 aa, synthetic construct
GGAGNDEVV

SEQ ID NO: 11254 - protein, 9 aa, synthetic construct
GGGGNDKLW

SEQ ID NO: 11255 - protein, 9 aa, synthetic construct
GGRGNDVIY

SEQ ID NO: 11256 - protein, 9 aa, synthetic construct
GGTGNDSVT

SEQ ID NO: 11257 - protein, 9 aa, synthetic construct
GGAGADTFG

SEQ ID NO: 11258 - protein, 9 aa, synthetic construct
GGDGNDFLR

SEQ ID NO: 11259 - protein, 9 aa, synthetic construct
GGGGNDRIW

SEQ ID NO: 11260 - protein, 9 aa, synthetic construct
GGRGNDMIN

SEQ ID NO: 11261 - protein, 9 aa, synthetic construct
GGTGNDSVL

SEQ ID NO: 11262 - protein, 9 aa, synthetic construct
GGRGNDVLL

SEQ ID NO: 11263 - protein, 9 aa, synthetic construct
GGRGNDVLN

SEQ ID NO: 11264 - protein, 9 aa, synthetic construct
GGTGNDWVE

SEQ ID NO: 11265 - protein, 9 aa, synthetic construct
GGLGADMLS

SEQ ID NO: 11266 - protein, 9 aa, synthetic construct
GGGGKDRLD

SEQ ID NO: 11267 - protein, 9 aa, synthetic construct
GGWGDDNLT

SEQ ID NO: 11268 - protein, 9 aa, synthetic construct
GGDGNDSIW

SEQ ID NO: 11269 - protein, 9 aa, synthetic construct
GGDGHDTLT

SEQ ID NO: 11270 - protein, 9 aa, synthetic construct
GGTGADLLA

SEQ ID NO: 11271 - protein, 9 aa, synthetic construct
GGAGQDTLR

SEQ ID NO: 11272 - protein, 9 aa, synthetic construct
GGEGTDSLA

SEQ ID NO: 11273 - protein, 9 aa, synthetic construct
GGTGNDSLQ

SEQ ID NO: 11274 - protein, 9 aa, synthetic construct
GGRGNDILK

SEQ ID NO: 11275 - protein, 9 aa, synthetic construct
GGIGDDSIA

SEQ ID NO: 11276 - protein, 9 aa, synthetic construct
GGTGNDSLM

SEQ ID NO: 11277 - protein, 9 aa, synthetic construct
GGTGNDSLK

SEQ ID NO: 11278 - protein, 9 aa, synthetic construct
GGEGNDALF

SEQ ID NO: 11279 - protein, 9 aa, synthetic construct
GGSGNDVIW

SEQ ID NO: 11280 - protein, 9 aa, synthetic construct
GGAGEDRLY

SEQ ID NO: 11281 - protein, 9 aa, synthetic construct
GGRGNDILS

SEQ ID NO: 11282 - protein, 9 aa, synthetic construct
GGDGDDLVL

SEQ ID NO: 11283 - protein, 9 aa, synthetic construct
GGTGNDSIN

SEQ ID NO: 11284 - protein, 9 aa, synthetic construct
GGDGVDTIQ

SEQ ID NO: 11285 - protein, 9 aa, synthetic construct
GGGGDDRLK

SEQ ID NO: 11286 - protein, 9 aa, synthetic construct
GGLGADQLF

SEQ ID NO: 11287 - protein, 9 aa, synthetic construct
GGAGADRYV

SEQ ID NO: 11288 - protein, 9 aa, synthetic construct
GGLGADQLG

SEQ ID NO: 11289 - protein, 9 aa, synthetic construct
GGLGRDTFV

SEQ ID NO: 11290 - protein, 9 aa, synthetic construct
GGLGADIIN

SEQ ID NO: 11291 - protein, 9 aa, synthetic construct
GGGGGDLLI

SEQ ID NO: 11292 - protein, 9 aa, synthetic construct
GGSGNDWIH

SEQ ID NO: 11293 - protein, 9 aa, synthetic construct
GGIGDDSLV

SEQ ID NO: 11294 - protein, 9 aa, synthetic construct
GGLGVDTMT

SEQ ID NO: 11295 - protein, 9 aa, synthetic construct
GGDGNDFLH

SEQ ID NO: 11296 - protein, 9 aa, synthetic construct
GGSGKDVFM

SEQ ID NO: 11297 - protein, 9 aa, synthetic construct
GGRGNDKLS

SEQ ID NO: 11298 - protein, 9 aa, synthetic construct
GGRGNDKLL

SEQ ID NO: 11299 - protein, 9 aa, synthetic construct
GGAGKDQID

SEQ ID NO: 11300 - protein, 9 aa, synthetic construct
GGAGVDTIN

SEQ ID NO: 11301 - protein, 9 aa, synthetic construct
GGAGADSFD

SEQ ID NO: 11302 - protein, 9 aa, synthetic construct
GGEGDDRII

SEQ ID NO: 11303 - protein, 9 aa, synthetic construct
GGIGDDSLN

SEQ ID NO: 11304 - protein, 9 aa, synthetic construct
GGAGQDTLK

SEQ ID NO: 11305 - protein, 9 aa, synthetic construct
GGIGDDSIL

SEQ ID NO: 11306 - protein, 9 aa, synthetic construct
GGIGTDIAD

SEQ ID NO: 11307 - protein, 9 aa, synthetic construct
GGWGDDLLS

SEQ ID NO: 11308 - protein, 9 aa, synthetic construct
GGLGADQFH

SEQ ID NO: 11309 - protein, 9 aa, synthetic construct
GGWGDDLLN

SEQ ID NO: 11310 - protein, 9 aa, synthetic construct
GGLGADQFV

SEQ ID NO: 11311 - protein, 9 aa, synthetic construct
GGDGNDYLA

SEQ ID NO: 11312 - protein, 9 aa, synthetic construct
GGSGNDVLG

SEQ ID NO: 11313 - protein, 9 aa, synthetic construct
GGGGADHLW

SEQ ID NO: 11314 - protein, 9 aa, synthetic construct
GGRGNDILY

SEQ ID NO: 11315 - protein, 9 aa, synthetic construct
GGIGTDALT

SEQ ID NO: 11316 - protein, 9 aa, synthetic construct
GGGGNDQLS

SEQ ID NO: 11317 - protein, 9 aa, synthetic construct
GGEGHDKLY

SEQ ID NO: 11318 - protein, 9 aa, synthetic construct
GGAGVDWLF

SEQ ID NO: 11319 - protein, 9 aa, synthetic construct
GGDGSDLLR

SEQ ID NO: 11320 - protein, 9 aa, synthetic construct
GGWGEDTFL

SEQ ID NO: 11321 - protein, 9 aa, synthetic construct
GGTGNDVAH

SEQ ID NO: 11322 - protein, 9 aa, synthetic construct
GGEGTDTLF

SEQ ID NO: 11323 - protein, 9 aa, synthetic construct
GGEGTDTLD

SEQ ID NO: 11324 - protein, 9 aa, synthetic construct
GGDGDDGIF

SEQ ID NO: 11325 - protein, 9 aa, synthetic construct
GGTGNDVFA

SEQ ID NO: 11326 - protein, 9 aa, synthetic construct
GGAGQDRLH

SEQ ID NO: 11327 - protein, 9 aa, synthetic construct
GGLGNDEIY

SEQ ID NO: 11328 - protein, 9 aa, synthetic construct
GGSGKDSFV

SEQ ID NO: 11329 - protein, 9 aa, synthetic construct
GGAGEDTVD

SEQ ID NO: 11330 - protein, 9 aa, synthetic construct
GGDGDDGIA

SEQ ID NO: 11331 - protein, 9 aa, synthetic construct
GGRGNDSLV

SEQ ID NO: 11332 - protein, 9 aa, synthetic construct
GGAGVDVFK

SEQ ID NO: 11333 - protein, 9 aa, synthetic construct
GGLGRDTLM

SEQ ID NO: 11334 - protein, 9 aa, synthetic construct
GGRGNDSLI

SEQ ID NO: 11335 - protein, 9 aa, synthetic construct
GGRGNDSLD

SEQ ID NO: 11336 - protein, 9 aa, synthetic construct
GGTGNDVIK

SEQ ID NO: 11337 - protein, 9 aa, synthetic construct
GGGGVDVFV

SEQ ID NO: 11338 - protein, 9 aa, synthetic construct
GGAGEDVIG

SEQ ID NO: 11339 - protein, 9 aa, synthetic construct
GGLGADLFV

SEQ ID NO: 11340 - protein, 9 aa, synthetic construct
GGAGADSLR

SEQ ID NO: 11341 - protein, 9 aa, synthetic construct
GGAGQDRLT

SEQ ID NO: 11342 - protein, 9 aa, synthetic construct
GGAGVDVLS

SEQ ID NO: 11343 - protein, 9 aa, synthetic construct
GGAGLDTIL

SEQ ID NO: 11344 - protein, 9 aa, synthetic construct
GGFGNDKID

SEQ ID NO: 11345 - protein, 9 aa, synthetic construct
GGGGKDQLK

SEQ ID NO: 11346 - protein, 9 aa, synthetic construct
GGDGNDVAH

SEQ ID NO: 11347 - protein, 9 aa, synthetic construct
GGSGKDRLE

SEQ ID NO: 11348 - protein, 9 aa, synthetic construct
GGSGKDRLS

SEQ ID NO: 11349 - protein, 9 aa, synthetic construct
GGAGVDVVV

SEQ ID NO: 11350 - protein, 9 aa, synthetic construct
GGRGNDTLQ

SEQ ID NO: 11351 - protein, 9 aa, synthetic construct
GGAGADSME

SEQ ID NO: 11352 - protein, 9 aa, synthetic construct
GGLGNDELQ

SEQ ID NO: 11353 - protein, 9 aa, synthetic construct
GGIGDDTLR

SEQ ID NO: 11354 - protein, 9 aa, synthetic construct
GGTGNDTIE

SEQ ID NO: 11355 - protein, 9 aa, synthetic construct
GGWGDDWLS

SEQ ID NO: 11356 - protein, 9 aa, synthetic construct
GGTGADLFI

SEQ ID NO: 11357 - protein, 9 aa, synthetic construct
GGKGDDVLA

SEQ ID NO: 11358 - protein, 9 aa, synthetic construct
GGEGDDIVN

SEQ ID NO: 11359 - protein, 9 aa, synthetic construct
GGTGNDTYH

SEQ ID NO: 11360 - protein, 9 aa, synthetic construct
GGDGNDFVL

SEQ ID NO: 11361 - protein, 9 aa, synthetic construct
GGLGADLFI

SEQ ID NO: 11362 - protein, 9 aa, synthetic construct
GGAGKDQLF

SEQ ID NO: 11363 - protein, 9 aa, synthetic construct
GGRGNDSIS

SEQ ID NO: 11364 - protein, 9 aa, synthetic construct
GGAGVDVAD

SEQ ID NO: 11365 - protein, 9 aa, synthetic construct
GGTGNDWLE

SEQ ID NO: 11366 - protein, 9 aa, synthetic construct
GGRGNDQLL

SEQ ID NO: 11367 - protein, 9 aa, synthetic construct
GGTGNDSYV

SEQ ID NO: 11368 - protein, 9 aa, synthetic construct
GGAGQDSLE

SEQ ID NO: 11369 - protein, 9 aa, synthetic construct
GGTGADKLS

SEQ ID NO: 11370 - protein, 9 aa, synthetic construct
GGAGQDSLL

SEQ ID NO: 11371 - protein, 9 aa, synthetic construct
GGGGNDKLL

SEQ ID NO: 11372 - protein, 9 aa, synthetic construct
GGGGVDVVT

SEQ ID NO: 11373 - protein, 9 aa, synthetic construct
GGEGDDIVT

SEQ ID NO: 11374 - protein, 9 aa, synthetic construct
GGIGSDYFV

SEQ ID NO: 11375 - protein, 9 aa, synthetic construct
GGEGEDRVF

SEQ ID NO: 11376 - protein, 9 aa, synthetic construct
GGWGGDELT

SEQ ID NO: 11377 - protein, 9 aa, synthetic construct
GGAGQDSLD

SEQ ID NO: 11378 - protein, 9 aa, synthetic construct
GGAGADSIY

SEQ ID NO: 11379 - protein, 9 aa, synthetic construct
GGGGQDRLD

SEQ ID NO: 11380 - protein, 9 aa, synthetic construct
GGRGNDQLD

SEQ ID NO: 11381 - protein, 9 aa, synthetic construct
GGEGDDVVE

SEQ ID NO: 11382 - protein, 9 aa, synthetic construct
GGRGNDQIS

SEQ ID NO: 11383 - protein, 9 aa, synthetic construct
GGAGIDKIF

SEQ ID NO: 11384 - protein, 9 aa, synthetic construct
GGSGNDVVY

SEQ ID NO: 11385 - protein, 9 aa, synthetic construct
GGAGEDTIN

SEQ ID NO: 11386 - protein, 9 aa, synthetic construct
GGAGADSIN

SEQ ID NO: 11387 - protein, 9 aa, synthetic construct
GGAGSDVIF

SEQ ID NO: 11388 - protein, 9 aa, synthetic construct
GGLGRDTLE

SEQ ID NO: 11389 - protein, 9 aa, synthetic construct
GGAGQDRLW

SEQ ID NO: 11390 - protein, 9 aa, synthetic construct
GGEGTDTLY

SEQ ID NO: 11391 - protein, 9 aa, synthetic construct
GGTGNDVIR

SEQ ID NO: 11392 - protein, 9 aa, synthetic construct
GGGGVDVLL

SEQ ID NO: 11393 - protein, 9 aa, synthetic construct
GGAGADSVE

SEQ ID NO: 11394 - protein, 9 aa, synthetic construct
GGIGDDTLG

SEQ ID NO: 11395 - protein, 9 aa, synthetic construct
GGMGEDTLV

SEQ ID NO: 11396 - protein, 9 aa, synthetic construct
GGAGNDEVS

SEQ ID NO: 11397 - protein, 9 aa, synthetic construct
GGRGNDRVR

SEQ ID NO: 11398 - protein, 9 aa, synthetic construct
GGDGSDLLI

SEQ ID NO: 11399 - protein, 9 aa, synthetic construct
GGLGNDFIL

SEQ ID NO: 11400 - protein, 9 aa, synthetic construct
GGTGNDTAA

SEQ ID NO: 11401 - protein, 9 aa, synthetic construct
GGRGNDRIY

SEQ ID NO: 11402 - protein, 9 aa, synthetic construct
GGTGNDVMR

SEQ ID NO: 11403 - protein, 9 aa, synthetic construct
GGRGNDTYR

SEQ ID NO: 11404 - protein, 9 aa, synthetic construct
GGAGVDTVI

SEQ ID NO: 11405 - protein, 9 aa, synthetic construct
GGTGNDVVN

SEQ ID NO: 11406 - protein, 9 aa, synthetic construct
GGGGDDRFY

SEQ ID NO: 11407 - protein, 9 aa, synthetic construct
GGDGDDNLS

SEQ ID NO: 11408 - protein, 9 aa, synthetic construct
GGDGVDTLL

SEQ ID NO: 11409 - protein, 9 aa, synthetic construct
GGIGDDTIR

SEQ ID NO: 11410 - protein, 9 aa, synthetic construct
GGTGNDSYW

SEQ ID NO: 11411 - protein, 9 aa, synthetic construct
GGGGDDQLA

SEQ ID NO: 11412 - protein, 9 aa, synthetic construct
GGGGADELR

SEQ ID NO: 11413 - protein, 9 aa, synthetic construct
GGAGEDVLV

SEQ ID NO: 11414 - protein, 9 aa, synthetic construct
GGFGNDLID

SEQ ID NO: 11415 - protein, 9 aa, synthetic construct
GGRGKDRLF

SEQ ID NO: 11416 - protein, 9 aa, synthetic construct
GGLGADRYV

SEQ ID NO: 11417 - protein, 9 aa, synthetic construct
GGPGLDVLD

SEQ ID NO: 11418 - protein, 9 aa, synthetic construct
GGTGNDRLW

SEQ ID NO: 11419 - protein, 9 aa, synthetic construct
GGFGDDSLN

SEQ ID NO: 11420 - protein, 9 aa, synthetic construct
GGAGRDDLA

SEQ ID NO: 11421 - protein, 9 aa, synthetic construct
GGRGKDMLD

SEQ ID NO: 11422 - protein, 9 aa, synthetic construct
GGGGRDVLN

SEQ ID NO: 11423 - protein, 9 aa, synthetic construct
GGSGNDTYT

SEQ ID NO: 11424 - protein, 9 aa, synthetic construct
GGMGGDVFQ

SEQ ID NO: 11425 - protein, 9 aa, synthetic construct
GGEGDDALA

SEQ ID NO: 11426 - protein, 9 aa, synthetic construct
GGDGQDRID

SEQ ID NO: 11427 - protein, 9 aa, synthetic construct
GGTGQDVFV

SEQ ID NO: 11428 - protein, 9 aa, synthetic construct
GGAGEDLVD

SEQ ID NO: 11429 - protein, 9 aa, synthetic construct
GGPGNDALY

SEQ ID NO: 11430 - protein, 9 aa, synthetic construct
GGPGDDTIN

SEQ ID NO: 11431 - protein, 9 aa, synthetic construct
GGDGNDELW

SEQ ID NO: 11432 - protein, 9 aa, synthetic construct
GGDGDDNLY

SEQ ID NO: 11433 - protein, 9 aa, synthetic construct
GGIGDDLIY

SEQ ID NO: 11434 - protein, 9 aa, synthetic construct
GGKGKDRIY

SEQ ID NO: 11435 - protein, 9 aa, synthetic construct
GGRGKDRLH

SEQ ID NO: 11436 - protein, 9 aa, synthetic construct
GGPGLDTLN

SEQ ID NO: 11437 - protein, 9 aa, synthetic construct
GGTGQDVLL

SEQ ID NO: 11438 - protein, 9 aa, synthetic construct
GGTGQDTLD

SEQ ID NO: 11439 - protein, 9 aa, synthetic construct
GGTGADIFK

SEQ ID NO: 11440 - protein, 9 aa, synthetic construct
GGEGDDILH

SEQ ID NO: 11441 - protein, 9 aa, synthetic construct
GGRGKDVLH

SEQ ID NO: 11442 - protein, 9 aa, synthetic construct
GGAGADTYI

SEQ ID NO: 11443 - protein, 9 aa, synthetic construct
GGLGADRMG

SEQ ID NO: 11444 - protein, 9 aa, synthetic construct
GGMGGDTYL

SEQ ID NO: 11445 - protein, 9 aa, synthetic construct
GGRGKDTLS

SEQ ID NO: 11446 - protein, 9 aa, synthetic construct
GGRGKDTLR

SEQ ID NO: 11447 - protein, 9 aa, synthetic construct
GGDGVDVLE

SEQ ID NO: 11448 - protein, 9 aa, synthetic construct
GGAGADTYY

SEQ ID NO: 11449 - protein, 9 aa, synthetic construct
GGPGDDTLE

SEQ ID NO: 11450 - protein, 9 aa, synthetic construct
GGAGRDALT

SEQ ID NO: 11451 - protein, 9 aa, synthetic construct
GGRGKDTLD

SEQ ID NO: 11452 - protein, 9 aa, synthetic construct
GGAGRDALV

SEQ ID NO: 11453 - protein, 9 aa, synthetic construct
GGAGQDKMF

SEQ ID NO: 11454 - protein, 9 aa, synthetic construct
GGAGVDRLI

SEQ ID NO: 11455 - protein, 9 aa, synthetic construct
GGGGKDTFI

SEQ ID NO: 11456 - protein, 9 aa, synthetic construct
GGTGNDRME

SEQ ID NO: 11457 - protein, 9 aa, synthetic construct
GGSGNDVAI

SEQ ID NO: 11458 - protein, 9 aa, synthetic construct
GGLGADELS

SEQ ID NO: 11459 - protein, 9 aa, synthetic construct
GGGGADIVS

SEQ ID NO: 11460 - protein, 9 aa, synthetic construct
GGVGVDRLY

SEQ ID NO: 11461 - protein, 9 aa, synthetic construct
GGGGIDILE

SEQ ID NO: 11462 - protein, 9 aa, synthetic construct
GGLGADDLL

SEQ ID NO: 11463 - protein, 9 aa, synthetic construct
GGDGNDELA

SEQ ID NO: 11464 - protein, 9 aa, synthetic construct
GGAGEDWID

SEQ ID NO: 11465 - protein, 9 aa, synthetic construct
GGTGNDTIW

SEQ ID NO: 11466 - protein, 9 aa, synthetic construct
GGDGGDELR

SEQ ID NO: 11467 - protein, 9 aa, synthetic construct
GGLGADTAI

SEQ ID NO: 11468 - protein, 9 aa, synthetic construct
GGSGSDRLD

SEQ ID NO: 11469 - protein, 9 aa, synthetic construct
GGTGNDRIV

SEQ ID NO: 11470 - protein, 9 aa, synthetic construct
GGSGSDRLN

SEQ ID NO: 11471 - protein, 9 aa, synthetic construct
GGWGNDQIY

SEQ ID NO: 11472 - protein, 9 aa, synthetic construct
GGRGHDVLI

SEQ ID NO: 11473 - protein, 9 aa, synthetic construct
GGAGVDQLF

SEQ ID NO: 11474 - protein, 9 aa, synthetic construct
GGSGSDRLQ

SEQ ID NO: 11475 - protein, 9 aa, synthetic construct
GGAGNDFIE

SEQ ID NO: 11476 - protein, 9 aa, synthetic construct
GGTGNDRIF

SEQ ID NO: 11477 - protein, 9 aa, synthetic construct
GGDGFDQIN

SEQ ID NO: 11478 - protein, 9 aa, synthetic construct
GGTGADGMW

SEQ ID NO: 11479 - protein, 9 aa, synthetic construct
GGRGHDTLI

SEQ ID NO: 11480 - protein, 9 aa, synthetic construct
GGEGHDALY

SEQ ID NO: 11481 - protein, 9 aa, synthetic construct
GGRGRDHLD

SEQ ID NO: 11482 - protein, 9 aa, synthetic construct
GGMGGDVMQ

SEQ ID NO: 11483 - protein, 9 aa, synthetic construct
GGGGNDIYV

SEQ ID NO: 11484 - protein, 9 aa, synthetic construct
GGNGADILT

SEQ ID NO: 11485 - protein, 9 aa, synthetic construct
GGAGNDEIQ

SEQ ID NO: 11486 - protein, 9 aa, synthetic construct
GGAGEDLLA

SEQ ID NO: 11487 - protein, 9 aa, synthetic construct
GGGGRDVLK

SEQ ID NO: 11488 - protein, 9 aa, synthetic construct
GGTGNDRLH

SEQ ID NO: 11489 - protein, 9 aa, synthetic construct
GGLGLDTLI

SEQ ID NO: 11490 - protein, 9 aa, synthetic construct
GGTGNDRIY

SEQ ID NO: 11491 - protein, 9 aa, synthetic construct
GGKGADTLV

SEQ ID NO: 11492 - protein, 9 aa, synthetic construct
GGRGKDALD

SEQ ID NO: 11493 - protein, 9 aa, synthetic construct
GGGGIDTLT

SEQ ID NO: 11494 - protein, 9 aa, synthetic construct
GGEGRDTLH

SEQ ID NO: 11495 - protein, 9 aa, synthetic construct
GGLGADSLV

SEQ ID NO: 11496 - protein, 9 aa, synthetic construct
GGSGSDRIY

SEQ ID NO: 11497 - protein, 9 aa, synthetic construct
GGTGADHLD

SEQ ID NO: 11498 - protein, 9 aa, synthetic construct
GGLGADDLY

SEQ ID NO: 11499 - protein, 9 aa, synthetic construct
GGAGEDLIT

SEQ ID NO: 11500 - protein, 9 aa, synthetic construct
GGAGIDLLN

SEQ ID NO: 11501 - protein, 9 aa, synthetic construct
GGAGVDQLV

SEQ ID NO: 11502 - protein, 9 aa, synthetic construct
GGEGEDTLK

SEQ ID NO: 11503 - protein, 9 aa, synthetic construct
GGAGRDELV

SEQ ID NO: 11504 - protein, 9 aa, synthetic construct
GGLGADSMS

SEQ ID NO: 11505 - protein, 9 aa, synthetic construct
GGIGDDIYY

SEQ ID NO: 11506 - protein, 9 aa, synthetic construct
GGGGNDLIK

SEQ ID NO: 11507 - protein, 9 aa, synthetic construct
GGEGTDKLF

SEQ ID NO: 11508 - protein, 9 aa, synthetic construct
GGRGKDVLT

SEQ ID NO: 11509 - protein, 9 aa, synthetic construct
GGAGKDMLY

SEQ ID NO: 11510 - protein, 9 aa, synthetic construct
GGTGNDRVY

SEQ ID NO: 11511 - protein, 9 aa, synthetic construct
GGRGNDELY

SEQ ID NO: 11512 - protein, 9 aa, synthetic construct
GGDGVDTID

SEQ ID NO: 11513 - protein, 9 aa, synthetic construct
GGLGADHMI

SEQ ID NO: 11514 - protein, 9 aa, synthetic construct
GGGGDDRLQ

SEQ ID NO: 11515 - protein, 9 aa, synthetic construct
GGRGNDEIS

SEQ ID NO: 11516 - protein, 9 aa, synthetic construct
GGEGHDILS

SEQ ID NO: 11517 - protein, 9 aa, synthetic construct
GGIGDDRLF

SEQ ID NO: 11518 - protein, 9 aa, synthetic construct
GGAGWDRLA

SEQ ID NO: 11519 - protein, 9 aa, synthetic construct
GGDGGDRFI

SEQ ID NO: 11520 - protein, 9 aa, synthetic construct
GGDGSDMLY

SEQ ID NO: 11521 - protein, 9 aa, synthetic construct
GGIGDDRLS

SEQ ID NO: 11522 - protein, 9 aa, synthetic construct
GGRGNDEID

SEQ ID NO: 11523 - protein, 9 aa, synthetic construct
GGAGQDVLA

SEQ ID NO: 11524 - protein, 9 aa, synthetic construct
GGNGNDLMY

SEQ ID NO: 11525 - protein, 9 aa, synthetic construct
GGAGQDVLD

SEQ ID NO: 11526 - protein, 9 aa, synthetic construct
GGAGVDSLN

SEQ ID NO: 11527 - protein, 9 aa, synthetic construct
GGAGQDVLL

SEQ ID NO: 11528 - protein, 9 aa, synthetic construct
GGGGHDVLF

SEQ ID NO: 11529 - protein, 9 aa, synthetic construct
GGGGADIFL

SEQ ID NO: 11530 - protein, 9 aa, synthetic construct
GGDGNDYIQ

SEQ ID NO: 11531 - protein, 9 aa, synthetic construct
GGRGNDEVV

SEQ ID NO: 11532 - protein, 9 aa, synthetic construct
GGDGVDTIF

SEQ ID NO: 11533 - protein, 9 aa, synthetic construct
GGEGADLID

SEQ ID NO: 11534 - protein, 9 aa, synthetic construct
GGEGADSLA

SEQ ID NO: 11535 - protein, 9 aa, synthetic construct
GGSGNDWLA

SEQ ID NO: 11536 - protein, 9 aa, synthetic construct
GGEGHDKLH

SEQ ID NO: 11537 - protein, 9 aa, synthetic construct
GGNGGDVVV

SEQ ID NO: 11538 - protein, 9 aa, synthetic construct
GGSGKDVLI

SEQ ID NO: 11539 - protein, 9 aa, synthetic construct
GGTGADLLF

SEQ ID NO: 11540 - protein, 9 aa, synthetic construct
GGDGSDMLI

SEQ ID NO: 11541 - protein, 9 aa, synthetic construct
GGRGNDGLF

SEQ ID NO: 11542 - protein, 9 aa, synthetic construct
GGDGVDTIH

SEQ ID NO: 11543 - protein, 9 aa, synthetic construct
GGAGEDRLD

SEQ ID NO: 11544 - protein, 9 aa, synthetic construct
GGRGNDFLN

SEQ ID NO: 11545 - protein, 9 aa, synthetic construct
GGTGADLLG

SEQ ID NO: 11546 - protein, 9 aa, synthetic construct
GGTGQDIFV

SEQ ID NO: 11547 - protein, 9 aa, synthetic construct
GGWGKDTLT

SEQ ID NO: 11548 - protein, 9 aa, synthetic construct
GGPGDDVLA

SEQ ID NO: 11549 - protein, 9 aa, synthetic construct
GGEGCDTIC

SEQ ID NO: 11550 - protein, 9 aa, synthetic construct
GGRGNDFLD

SEQ ID NO: 11551 - protein, 9 aa, synthetic construct
GGAGVDTAA

SEQ ID NO: 11552 - protein, 9 aa, synthetic construct
GGTGQDILF

SEQ ID NO: 11553 - protein, 9 aa, synthetic construct
GGEGHDRIF

SEQ ID NO: 11554 - protein, 9 aa, synthetic construct
GGWGADTLH

SEQ ID NO: 11555 - protein, 9 aa, synthetic construct
GGDGIDRLS

SEQ ID NO: 11556 - protein, 9 aa, synthetic construct
GGFGNDVLS

SEQ ID NO: 11557 - protein, 9 aa, synthetic construct
GGLGADRLW

SEQ ID NO: 11558 - protein, 9 aa, synthetic construct
GGEGHDRLN

SEQ ID NO: 11559 - protein, 9 aa, synthetic construct
GGAGEDQID

SEQ ID NO: 11560 - protein, 9 aa, synthetic construct
GGRGLDTLN

SEQ ID NO: 11561 - protein, 9 aa, synthetic construct
GGEGHDILF

SEQ ID NO: 11562 - protein, 9 aa, synthetic construct
GGAGRDAFI

SEQ ID NO: 11563 - protein, 9 aa, synthetic construct
GGNGADKLD

SEQ ID NO: 11564 - protein, 9 aa, synthetic construct
GGAGIDLAS

SEQ ID NO: 11565 - protein, 9 aa, synthetic construct
GGNGHDRIY

SEQ ID NO: 11566 - protein, 9 aa, synthetic construct
GGDGDDFLL

SEQ ID NO: 11567 - protein, 9 aa, synthetic construct
GGAGADTVW

SEQ ID NO: 11568 - protein, 9 aa, synthetic construct
GGAGNDELG

SEQ ID NO: 11569 - protein, 9 aa, synthetic construct
GGLGMDQLS

SEQ ID NO: 11570 - protein, 9 aa, synthetic construct
GGEGNDALL

SEQ ID NO: 11571 - protein, 9 aa, synthetic construct
GGLGADRLN

SEQ ID NO: 11572 - protein, 9 aa, synthetic construct
GGPGDDTLS

SEQ ID NO: 11573 - protein, 9 aa, synthetic construct
GGTGNDRMN

SEQ ID NO: 11574 - protein, 9 aa, synthetic construct
GGKGADTMA

SEQ ID NO: 11575 - protein, 9 aa, synthetic construct
GGAGKDRAD

SEQ ID NO: 11576 - protein, 9 aa, synthetic construct
GGDGNDSAY

SEQ ID NO: 11577 - protein, 9 aa, synthetic construct
GGAGKDRFI

SEQ ID NO: 11578 - protein, 9 aa, synthetic construct
GGLGTDTAA

SEQ ID NO: 11579 - protein, 9 aa, synthetic construct
GGWGNDILV

SEQ ID NO: 11580 - protein, 9 aa, synthetic construct
GGTGNDRMV

SEQ ID NO: 11581 - protein, 9 aa, synthetic construct
GGRGNDAYA

SEQ ID NO: 11582 - protein, 9 aa, synthetic construct
GGTGQDRFV

SEQ ID NO: 11583 - protein, 9 aa, synthetic construct
GGSGKDVLN

SEQ ID NO: 11584 - protein, 9 aa, synthetic construct
GGPGKDELY

SEQ ID NO: 11585 - protein, 9 aa, synthetic construct
GGAGQDVLS

SEQ ID NO: 11586 - protein, 9 aa, synthetic construct
GGDGDDLVN

SEQ ID NO: 11587 - protein, 9 aa, synthetic construct
GGWGADKMF

SEQ ID NO: 11588 - protein, 9 aa, synthetic construct
GGGGADIFM

SEQ ID NO: 11589 - protein, 9 aa, synthetic construct
GGIGDDQLF

SEQ ID NO: 11590 - protein, 9 aa, synthetic construct
GGDGSDNLS

SEQ ID NO: 11591 - protein, 9 aa, synthetic construct
GGIGDDQIN

SEQ ID NO: 11592 - protein, 9 aa, synthetic construct
GGAGWDTAD

SEQ ID NO: 11593 - protein, 9 aa, synthetic construct
GGNGADKLF

SEQ ID NO: 11594 - protein, 9 aa, synthetic construct
GGTGADIIV

SEQ ID NO: 11595 - protein, 9 aa, synthetic construct
GGLGNDGYY

SEQ ID NO: 11596 - protein, 9 aa, synthetic construct
GGGGADIIE

SEQ ID NO: 11597 - protein, 9 aa, synthetic construct
GGAGADTVN

SEQ ID NO: 11598 - protein, 9 aa, synthetic construct
GGLGADRLA

SEQ ID NO: 11599 - protein, 9 aa, synthetic construct
GGAGADRMQ

SEQ ID NO: 11600 - protein, 9 aa, synthetic construct
GGLGNDHIE

SEQ ID NO: 11601 - protein, 9 aa, synthetic construct
GGEGNDWLY

SEQ ID NO: 11602 - protein, 9 aa, synthetic construct
GGRGMDKLS

SEQ ID NO: 11603 - protein, 9 aa, synthetic construct
GGGGRDVMD

SEQ ID NO: 11604 - protein, 9 aa, synthetic construct
GGRGNDRID

SEQ ID NO: 11605 - protein, 9 aa, synthetic construct
GGRGDDILN

SEQ ID NO: 11606 - protein, 9 aa, synthetic construct
GGFGNDSIR

SEQ ID NO: 11607 - protein, 9 aa, synthetic construct
GGSGNDIYI

SEQ ID NO: 11608 - protein, 9 aa, synthetic construct
GGQGDDDLN

SEQ ID NO: 11609 - protein, 9 aa, synthetic construct
GGGGADTMN

SEQ ID NO: 11610 - protein, 9 aa, synthetic construct
GGNGNDALT

SEQ ID NO: 11611 - protein, 9 aa, synthetic construct
GGQGNDMLV

SEQ ID NO: 11612 - protein, 9 aa, synthetic construct
GGGGNDSIF

SEQ ID NO: 11613 - protein, 9 aa, synthetic construct
GGSGNDIYQ

SEQ ID NO: 11614 - protein, 9 aa, synthetic construct
GGSGNDIYR

SEQ ID NO: 11615 - protein, 9 aa, synthetic construct
GGQGDDELH

SEQ ID NO: 11616 - protein, 9 aa, synthetic construct
GGDGDDVIW

SEQ ID NO: 11617 - protein, 9 aa, synthetic construct
GGLGSDRLT

SEQ ID NO: 11618 - protein, 9 aa, synthetic construct
GGGGNDAID

SEQ ID NO: 11619 - protein, 9 aa, synthetic construct
GGAGIDTLL

SEQ ID NO: 11620 - protein, 9 aa, synthetic construct
GGVGDDILL

SEQ ID NO: 11621 - protein, 9 aa, synthetic construct
GGEGFDTLV

SEQ ID NO: 11622 - protein, 9 aa, synthetic construct
GGVGDDILT

SEQ ID NO: 11623 - protein, 9 aa, synthetic construct
GGMGQDLIL

SEQ ID NO: 11624 - protein, 9 aa, synthetic construct
GGQGDDFIA

SEQ ID NO: 11625 - protein, 9 aa, synthetic construct
GGQGNDLLQ

SEQ ID NO: 11626 - protein, 9 aa, synthetic construct
GGQGNDLLK

SEQ ID NO: 11627 - protein, 9 aa, synthetic construct
GGSGNDKLA

SEQ ID NO: 11628 - protein, 9 aa, synthetic construct
GGVGDDKLF

SEQ ID NO: 11629 - protein, 9 aa, synthetic construct
GGQGNDLIY

SEQ ID NO: 11630 - protein, 9 aa, synthetic construct
GGLGGDELT

SEQ ID NO: 11631 - protein, 9 aa, synthetic construct
GGAGSDLYV

SEQ ID NO: 11632 - protein, 9 aa, synthetic construct
GGQGNDNIN

SEQ ID NO: 11633 - protein, 9 aa, synthetic construct
GGQGNDELL

SEQ ID NO: 11634 - protein, 9 aa, synthetic construct
GGSGNDIVD

SEQ ID NO: 11635 - protein, 9 aa, synthetic construct
GGDGTDILD

SEQ ID NO: 11636 - protein, 9 aa, synthetic construct
GGAGDDNAG

SEQ ID NO: 11637 - protein, 9 aa, synthetic construct
GGVGDDDLS

SEQ ID NO: 11638 - protein, 9 aa, synthetic construct
GGAGSDLLT

SEQ ID NO: 11639 - protein, 9 aa, synthetic construct
GGEGFDTIR

SEQ ID NO: 11640 - protein, 9 aa, synthetic construct
GGAGDDFIH

SEQ ID NO: 11641 - protein, 9 aa, synthetic construct
GGLGQDVLT

SEQ ID NO: 11642 - protein, 9 aa, synthetic construct
GGAGIDTLK

SEQ ID NO: 11643 - protein, 9 aa, synthetic construct
GGFGNDSLD

SEQ ID NO: 11644 - protein, 9 aa, synthetic construct
GGGGIDRLD

SEQ ID NO: 11645 - protein, 9 aa, synthetic construct
GGQGNDQLE

SEQ ID NO: 11646 - protein, 9 aa, synthetic construct
GGQGDDALF

SEQ ID NO: 11647 - protein, 9 aa, synthetic construct
GGSGNDIVN

SEQ ID NO: 11648 - protein, 9 aa, synthetic construct
GGQGDDALS

SEQ ID NO: 11649 - protein, 9 aa, synthetic construct
GGQGDDALY

SEQ ID NO: 11650 - protein, 9 aa, synthetic construct
GGLGGDKIN

SEQ ID NO: 11651 - protein, 9 aa, synthetic construct
GGQGDDAYY

SEQ ID NO: 11652 - protein, 9 aa, synthetic construct
GGGGADTME

SEQ ID NO: 11653 - protein, 9 aa, synthetic construct
GGQGDDDIN

SEQ ID NO: 11654 - protein, 9 aa, synthetic construct
GGLGGDILT

SEQ ID NO: 11655 - protein, 9 aa, synthetic construct
GGQGNDNLT

SEQ ID NO: 11656 - protein, 9 aa, synthetic construct
GGVGDDFLL

SEQ ID NO: 11657 - protein, 9 aa, synthetic construct
GGDGDDDIT

SEQ ID NO: 11658 - protein, 9 aa, synthetic construct
GGAGTDEME

SEQ ID NO: 11659 - protein, 9 aa, synthetic construct
GGVGNDILM

SEQ ID NO: 11660 - protein, 9 aa, synthetic construct
GGAGTDDLS

SEQ ID NO: 11661 - protein, 9 aa, synthetic construct
GGSGNDQVF

SEQ ID NO: 11662 - protein, 9 aa, synthetic construct
GGNGDDLIF

SEQ ID NO: 11663 - protein, 9 aa, synthetic construct
GGAGDDLVS

SEQ ID NO: 11664 - protein, 9 aa, synthetic construct
GGAGSDNLI

SEQ ID NO: 11665 - protein, 9 aa, synthetic construct
GGEGGDLLM

SEQ ID NO: 11666 - protein, 9 aa, synthetic construct
GGSGNDKLW

SEQ ID NO: 11667 - protein, 9 aa, synthetic construct
GGAGDDLVL

SEQ ID NO: 11668 - protein, 9 aa, synthetic construct
GGAGDDLVI

SEQ ID NO: 11669 - protein, 9 aa, synthetic construct
GGVGDDNLS

SEQ ID NO: 11670 - protein, 9 aa, synthetic construct
GGVGDDNMG

SEQ ID NO: 11671 - protein, 9 aa, synthetic construct
GGDGDDVYV

SEQ ID NO: 11672 - protein, 9 aa, synthetic construct
GGAGSDNLT

SEQ ID NO: 11673 - protein, 9 aa, synthetic construct
GGQGDDILQ

SEQ ID NO: 11674 - protein, 9 aa, synthetic construct
GGDGDDVYL

SEQ ID NO: 11675 - protein, 9 aa, synthetic construct
GGGGGDTLE

SEQ ID NO: 11676 - protein, 9 aa, synthetic construct
GGVGDDQLF

SEQ ID NO: 11677 - protein, 9 aa, synthetic construct
GGVGDDQLS

SEQ ID NO: 11678 - protein, 9 aa, synthetic construct
GGAGDDLMY

SEQ ID NO: 11679 - protein, 9 aa, synthetic construct
GGEGSDRFV

SEQ ID NO: 11680 - protein, 9 aa, synthetic construct
GGDGDDAIE

SEQ ID NO: 11681 - protein, 9 aa, synthetic construct
GGKGGDLLH

SEQ ID NO: 11682 - protein, 9 aa, synthetic construct
GGGGNDALA

SEQ ID NO: 11683 - protein, 9 aa, synthetic construct
GGLGDDTVF

SEQ ID NO: 11684 - protein, 9 aa, synthetic construct
GGEGGDLLD

SEQ ID NO: 11685 - protein, 9 aa, synthetic construct
GGDGPDWVV

SEQ ID NO: 11686 - protein, 9 aa, synthetic construct
GGLGRDILS

SEQ ID NO: 11687 - protein, 9 aa, synthetic construct
GGVGDDMLW

SEQ ID NO: 11688 - protein, 9 aa, synthetic construct
GGDGKDSLF

SEQ ID NO: 11689 - protein, 9 aa, synthetic construct
GGGGIDRLL

SEQ ID NO: 11690 - protein, 9 aa, synthetic construct
GGSGNDKLR

SEQ ID NO: 11691 - protein, 9 aa, synthetic construct
GGLGDDTII

SEQ ID NO: 11692 - protein, 9 aa, synthetic construct
GGVGNDILA

SEQ ID NO: 11693 - protein, 9 aa, synthetic construct
GGSGVDQIF

SEQ ID NO: 11694 - protein, 9 aa, synthetic construct
GGAGIDTMT

SEQ ID NO: 11695 - protein, 9 aa, synthetic construct
GGLGDDTIQ

SEQ ID NO: 11696 - protein, 9 aa, synthetic construct
GGEGADQLI

SEQ ID NO: 11697 - protein, 9 aa, synthetic construct
GGVGNDIIE

SEQ ID NO: 11698 - protein, 9 aa, synthetic construct
GGNGNDAIY

SEQ ID NO: 11699 - protein, 9 aa, synthetic construct
GGGGADTVD

SEQ ID NO: 11700 - protein, 9 aa, synthetic construct
GGDGKDRLW

SEQ ID NO: 11701 - protein, 9 aa, synthetic construct
GGLGDDTIW

SEQ ID NO: 11702 - protein, 9 aa, synthetic construct
GGSGTDRAI

SEQ ID NO: 11703 - protein, 9 aa, synthetic construct
GGAGDDLYY

SEQ ID NO: 11704 - protein, 9 aa, synthetic construct
GGVGDDLLA

SEQ ID NO: 11705 - protein, 9 aa, synthetic construct
GGAGDDLYV

SEQ ID NO: 11706 - protein, 9 aa, synthetic construct
GGAGSDNID

SEQ ID NO: 11707 - protein, 9 aa, synthetic construct
GGVGDDLLF

SEQ ID NO: 11708 - protein, 9 aa, synthetic construct
GGGGNDSII

SEQ ID NO: 11709 - protein, 9 aa, synthetic construct
GGMGNDQLH

SEQ ID NO: 11710 - protein, 9 aa, synthetic construct
GGAGDDLYI

SEQ ID NO: 11711 - protein, 9 aa, synthetic construct
GGAGDDLYF

SEQ ID NO: 11712 - protein, 9 aa, synthetic construct
GGKGEDTLT

SEQ ID NO: 11713 - protein, 9 aa, synthetic construct
GGDGNDTML

SEQ ID NO: 11714 - protein, 9 aa, synthetic construct
GGAGTDGMD

SEQ ID NO: 11715 - protein, 9 aa, synthetic construct
GGDGQDCLV

SEQ ID NO: 11716 - protein, 9 aa, synthetic construct
GGQGNDRLL

SEQ ID NO: 11717 - protein, 9 aa, synthetic construct
GGGGRDRLW

SEQ ID NO: 11718 - protein, 9 aa, synthetic construct
GGVGADRLS

SEQ ID NO: 11719 - protein, 9 aa, synthetic construct
GGDGLDTLR

SEQ ID NO: 11720 - protein, 9 aa, synthetic construct
GGKGGDTLS

SEQ ID NO: 11721 - protein, 9 aa, synthetic construct
GGQGADSLY

SEQ ID NO: 11722 - protein, 9 aa, synthetic construct
GGEGFDTAD

SEQ ID NO: 11723 - protein, 9 aa, synthetic construct
GGVGADRMI

SEQ ID NO: 11724 - protein, 9 aa, synthetic construct
GGEGNDDLA

SEQ ID NO: 11725 - protein, 9 aa, synthetic construct
GGQGNDVLA

SEQ ID NO: 11726 - protein, 9 aa, synthetic construct
GGLGGDTLD

SEQ ID NO: 11727 - protein, 9 aa, synthetic construct
GGQGADTAY

SEQ ID NO: 11728 - protein, 9 aa, synthetic construct
GGNGNDDLY

SEQ ID NO: 11729 - protein, 9 aa, synthetic construct
GGVGADSLL

SEQ ID NO: 11730 - protein, 9 aa, synthetic construct
GGGGIDTFI

SEQ ID NO: 11731 - protein, 9 aa, synthetic construct
GGQGADTIE

SEQ ID NO: 11732 - protein, 9 aa, synthetic construct
GGSGNDIFY

SEQ ID NO: 11733 - protein, 9 aa, synthetic construct
GGSGNDIIA

SEQ ID NO: 11734 - protein, 9 aa, synthetic construct
GGVGADSLT

SEQ ID NO: 11735 - protein, 9 aa, synthetic construct
GGSGNDRIQ

SEQ ID NO: 11736 - protein, 9 aa, synthetic construct
GGVGNDMLN

SEQ ID NO: 11737 - protein, 9 aa, synthetic construct
GGQGNDTVL

SEQ ID NO: 11738 - protein, 9 aa, synthetic construct
GGVGADSMV

SEQ ID NO: 11739 - protein, 9 aa, synthetic construct
GGVGADTAI

SEQ ID NO: 11740 - protein, 9 aa, synthetic construct
GGLGDDSIL

SEQ ID NO: 11741 - protein, 9 aa, synthetic construct
GGGGRDRLV

SEQ ID NO: 11742 - protein, 9 aa, synthetic construct
GGFGDDVIY

SEQ ID NO: 11743 - protein, 9 aa, synthetic construct
GGQGNDVLY

SEQ ID NO: 11744 - protein, 9 aa, synthetic construct
GGLGGDTLL

SEQ ID NO: 11745 - protein, 9 aa, synthetic construct
GGNGNDEID

SEQ ID NO: 11746 - protein, 9 aa, synthetic construct
GGLGDDRLL

SEQ ID NO: 11747 - protein, 9 aa, synthetic construct
GGGGADTIF

SEQ ID NO: 11748 - protein, 9 aa, synthetic construct
GGQGADRLH

SEQ ID NO: 11749 - protein, 9 aa, synthetic construct
GGLGDDRLQ

SEQ ID NO: 11750 - protein, 9 aa, synthetic construct
GGLGDDRLS

SEQ ID NO: 11751 - protein, 9 aa, synthetic construct
GGQGNDYLY

SEQ ID NO: 11752 - protein, 9 aa, synthetic construct
GGAGKDFLV

SEQ ID NO: 11753 - protein, 9 aa, synthetic construct
GGGGEDVVD

SEQ ID NO: 11754 - protein, 9 aa, synthetic construct
GGQGNDYLD

SEQ ID NO: 11755 - protein, 9 aa, synthetic construct
GGQGADRMT

SEQ ID NO: 11756 - protein, 9 aa, synthetic construct
GGAGSDIVY

SEQ ID NO: 11757 - protein, 9 aa, synthetic construct
GGSGNDRLR

SEQ ID NO: 11758 - protein, 9 aa, synthetic construct
GGQGADSFV

SEQ ID NO: 11759 - protein, 9 aa, synthetic construct
GGDGDDWLH

SEQ ID NO: 11760 - protein, 9 aa, synthetic construct
GGDGPDLIG

SEQ ID NO: 11761 - protein, 9 aa, synthetic construct
GGAGSDIYV

SEQ ID NO: 11762 - protein, 9 aa, synthetic construct
GGFGDDVIS

SEQ ID NO: 11763 - protein, 9 aa, synthetic construct
GGHGDDTYV

SEQ ID NO: 11764 - protein, 9 aa, synthetic construct
GGAGMDTLD

SEQ ID NO: 11765 - protein, 9 aa, synthetic construct
GGQGNDVYY

SEQ ID NO: 11766 - protein, 9 aa, synthetic construct
GGQGNDVYV

SEQ ID NO: 11767 - protein, 9 aa, synthetic construct
GGSGVDTVD

SEQ ID NO: 11768 - protein, 9 aa, synthetic construct
GGAGDDEMT

SEQ ID NO: 11769 - protein, 9 aa, synthetic construct
GGQGNDTMF

SEQ ID NO: 11770 - protein, 9 aa, synthetic construct
GGEGNDTIR

SEQ ID NO: 11771 - protein, 9 aa, synthetic construct
GGAGSDLLM

SEQ ID NO: 11772 - protein, 9 aa, synthetic construct
GGNGDDTLH

SEQ ID NO: 11773 - protein, 9 aa, synthetic construct
GGSGNDILK

SEQ ID NO: 11774 - protein, 9 aa, synthetic construct
GGLGGDSLH

SEQ ID NO: 11775 - protein, 9 aa, synthetic construct
GGAGSDLIS

SEQ ID NO: 11776 - protein, 9 aa, synthetic construct
GGAGSDLIV

SEQ ID NO: 11777 - protein, 9 aa, synthetic construct
GGVGADVLS

SEQ ID NO: 11778 - protein, 9 aa, synthetic construct
GGLGDDSLH

SEQ ID NO: 11779 - protein, 9 aa, synthetic construct
GGDGDDMLN

SEQ ID NO: 11780 - protein, 9 aa, synthetic construct
GGAGTDIAD

SEQ ID NO: 11781 - protein, 9 aa, synthetic construct
GGNGNDDLE

SEQ ID NO: 11782 - protein, 9 aa, synthetic construct
GGEGADQLS

SEQ ID NO: 11783 - protein, 9 aa, synthetic construct
GGVGNDLLK

SEQ ID NO: 11784 - protein, 9 aa, synthetic construct
GGAGTDHLW

SEQ ID NO: 11785 - protein, 9 aa, synthetic construct
GGSGNDIIF

SEQ ID NO: 11786 - protein, 9 aa, synthetic construct
GGGGNDSMH

SEQ ID NO: 11787 - protein, 9 aa, synthetic construct
GGQGNDSIL

SEQ ID NO: 11788 - protein, 9 aa, synthetic construct
GGSGNDILW

SEQ ID NO: 11789 - protein, 9 aa, synthetic construct
GGQGNDSIF

SEQ ID NO: 11790 - protein, 9 aa, synthetic construct
GGEGNDDLG

SEQ ID NO: 11791 - protein, 9 aa, synthetic construct
GGQGADVLR

SEQ ID NO: 11792 - protein, 9 aa, synthetic construct
GGSGNDIMA

SEQ ID NO: 11793 - protein, 9 aa, synthetic construct
GGEGADQLR

SEQ ID NO: 11794 - protein, 9 aa, synthetic construct
GGAGLDVLR

SEQ ID NO: 11795 - protein, 9 aa, synthetic construct
GGAGTDHLI

SEQ ID NO: 11796 - protein, 9 aa, synthetic construct
GGAGTDHLD

SEQ ID NO: 11797 - protein, 9 aa, synthetic construct
GGQGADTYL

SEQ ID NO: 11798 - protein, 9 aa, synthetic construct
GGEGDDFLD

SEQ ID NO: 11799 - protein, 9 aa, synthetic construct
GGSGTDMIY

SEQ ID NO: 11800 - protein, 9 aa, synthetic construct
GGDGFDTVS

SEQ ID NO: 11801 - protein, 9 aa, synthetic construct
GGNGNDDLR

SEQ ID NO: 11802 - protein, 9 aa, synthetic construct
GGVGADTIN

SEQ ID NO: 11803 - protein, 9 aa, synthetic construct
GGMGNDLMT

SEQ ID NO: 11804 - protein, 9 aa, synthetic construct
GGVGADTIY

SEQ ID NO: 11805 - protein, 9 aa, synthetic construct
GGSGNDIII

SEQ ID NO: 11806 - protein, 9 aa, synthetic construct
GGHGDDYAE

SEQ ID NO: 11807 - protein, 9 aa, synthetic construct
GGSGVDTMI

SEQ ID NO: 11808 - protein, 9 aa, synthetic construct
GGEGSDSLY

SEQ ID NO: 11809 - protein, 9 aa, synthetic construct
GGVGADTML

SEQ ID NO: 11810 - protein, 9 aa, synthetic construct
GGQGADTMI

SEQ ID NO: 11811 - protein, 9 aa, synthetic construct
GGDGKDLYI

SEQ ID NO: 11812 - protein, 9 aa, synthetic construct
GGFGDDVLD

SEQ ID NO: 11813 - protein, 9 aa, synthetic construct
GGQGADTMS

SEQ ID NO: 11814 - protein, 9 aa, synthetic construct
GGQGADTMT

SEQ ID NO: 11815 - protein, 9 aa, synthetic construct
GGDGTDFAY

SEQ ID NO: 11816 - protein, 9 aa, synthetic construct
GGAGTDILA

SEQ ID NO: 11817 - protein, 9 aa, synthetic construct
GGVGADVFK

SEQ ID NO: 11818 - protein, 9 aa, synthetic construct
GGEGNDTIV

SEQ ID NO: 11819 - protein, 9 aa, synthetic construct
GGDGDDVIH

SEQ ID NO: 11820 - protein, 9 aa, synthetic construct
GGVGADVFV

SEQ ID NO: 11821 - protein, 9 aa, synthetic construct
GGQGNDTFY

SEQ ID NO: 11822 - protein, 9 aa, synthetic construct
GGVGNDLMQ

SEQ ID NO: 11823 - protein, 9 aa, synthetic construct
GGAGIDTIK

SEQ ID NO: 11824 - protein, 9 aa, synthetic construct
GGQGDDIYI

SEQ ID NO: 11825 - protein, 9 aa, synthetic construct
GGLGDDTVN

SEQ ID NO: 11826 - protein, 9 aa, synthetic construct
GGHGADTLL

SEQ ID NO: 11827 - protein, 9 aa, synthetic construct
GGAGDDHLR

SEQ ID NO: 11828 - protein, 9 aa, synthetic construct
GGAGSDVLS

SEQ ID NO: 11829 - protein, 9 aa, synthetic construct
GGAGDDKLA

SEQ ID NO: 11830 - protein, 9 aa, synthetic construct
GGAGDDKIY

SEQ ID NO: 11831 - protein, 9 aa, synthetic construct
GGDGDDVVK

SEQ ID NO: 11832 - protein, 9 aa, synthetic construct
GGAGDDKIT

SEQ ID NO: 11833 - protein, 9 aa, synthetic construct
GGSGVDAFS

SEQ ID NO: 11834 - protein, 9 aa, synthetic construct
GGNGDDLVD

SEQ ID NO: 11835 - protein, 9 aa, synthetic construct
GGEGSDLYV

SEQ ID NO: 11836 - protein, 9 aa, synthetic construct
GGEGNDELD

SEQ ID NO: 11837 - protein, 9 aa, synthetic construct
GGDGFDFID

SEQ ID NO: 11838 - protein, 9 aa, synthetic construct
GGKGADKFV

SEQ ID NO: 11839 - protein, 9 aa, synthetic construct
GGSGNDNLN

SEQ ID NO: 11840 - protein, 9 aa, synthetic construct
GGVGEDVLI

SEQ ID NO: 11841 - protein, 9 aa, synthetic construct
GGGGGDTIT

SEQ ID NO: 11842 - protein, 9 aa, synthetic construct
GGLGVDILN

SEQ ID NO: 11843 - protein, 9 aa, synthetic construct
GGQGDDTLF

SEQ ID NO: 11844 - protein, 9 aa, synthetic construct
GGMGNDTLY

SEQ ID NO: 11845 - protein, 9 aa, synthetic construct
GGVGGDRFV

SEQ ID NO: 11846 - protein, 9 aa, synthetic construct
GGHGNDILT

SEQ ID NO: 11847 - protein, 9 aa, synthetic construct
GGSGNDNLF

SEQ ID NO: 11848 - protein, 9 aa, synthetic construct
GGEGKDTLF

SEQ ID NO: 11849 - protein, 9 aa, synthetic construct
GGSGNDLYV

SEQ ID NO: 11850 - protein, 9 aa, synthetic construct
GGAGSDTLW

SEQ ID NO: 11851 - protein, 9 aa, synthetic construct
GGLGDDYLS

SEQ ID NO: 11852 - protein, 9 aa, synthetic construct
GGNGLDTLL

SEQ ID NO: 11853 - protein, 9 aa, synthetic construct
GGGGADVVF

SEQ ID NO: 11854 - protein, 9 aa, synthetic construct
GGDGDDVYI

SEQ ID NO: 11855 - protein, 9 aa, synthetic construct
GGSGNDNVT

SEQ ID NO: 11856 - protein, 9 aa, synthetic construct
GGAGLDYLD

SEQ ID NO: 11857 - protein, 9 aa, synthetic construct
GGVGEDFVD

SEQ ID NO: 11858 - protein, 9 aa, synthetic construct
GGAGMDRLI

SEQ ID NO: 11859 - protein, 9 aa, synthetic construct
GGQGHDRLY

SEQ ID NO: 11860 - protein, 9 aa, synthetic construct
GGGGRDLLT

SEQ ID NO: 11861 - protein, 9 aa, synthetic construct
GGGGGDTIV

SEQ ID NO: 11862 - protein, 9 aa, synthetic construct
GGGGADVMD

SEQ ID NO: 11863 - protein, 9 aa, synthetic construct
GGGGNDAVI

SEQ ID NO: 11864 - protein, 9 aa, synthetic construct
GGQGDDSIL

SEQ ID NO: 11865 - protein, 9 aa, synthetic construct
GGGGFDQLR

SEQ ID NO: 11866 - protein, 9 aa, synthetic construct
GGNGLDTLV

SEQ ID NO: 11867 - protein, 9 aa, synthetic construct
GGDGPDTLI

SEQ ID NO: 11868 - protein, 9 aa, synthetic construct
GGAGDDKLI

SEQ ID NO: 11869 - protein, 9 aa, synthetic construct
GGLGEDTLT

SEQ ID NO: 11870 - protein, 9 aa, synthetic construct
GGGGNDELF

SEQ ID NO: 11871 - protein, 9 aa, synthetic construct
GGSGTDTFV

SEQ ID NO: 11872 - protein, 9 aa, synthetic construct
GGAGDDHIS

SEQ ID NO: 11873 - protein, 9 aa, synthetic construct
GGMGNDTYV

SEQ ID NO: 11874 - protein, 9 aa, synthetic construct
GGNGDDLLQ

SEQ ID NO: 11875 - protein, 9 aa, synthetic construct
GGEGADNLY

SEQ ID NO: 11876 - protein, 9 aa, synthetic construct
GGDGFDEIK

SEQ ID NO: 11877 - protein, 9 aa, synthetic construct
GGEGDDEIV

SEQ ID NO: 11878 - protein, 9 aa, synthetic construct
GGEGGDIFK

SEQ ID NO: 11879 - protein, 9 aa, synthetic construct
GGDGDDALL

SEQ ID NO: 11880 - protein, 9 aa, synthetic construct
GGQGDDTLW

SEQ ID NO: 11881 - protein, 9 aa, synthetic construct
GGNGLDILV

SEQ ID NO: 11882 - protein, 9 aa, synthetic construct
GGVGKDRLY

SEQ ID NO: 11883 - protein, 9 aa, synthetic construct
GGFGNDRLD

SEQ ID NO: 11884 - protein, 9 aa, synthetic construct
GGAGDDIMI

SEQ ID NO: 11885 - protein, 9 aa, synthetic construct
GGVGKDELY

SEQ ID NO: 11886 - protein, 9 aa, synthetic construct
GGQGDDVIH

SEQ ID NO: 11887 - protein, 9 aa, synthetic construct
GGKGFDSLV

SEQ ID NO: 11888 - protein, 9 aa, synthetic construct
GGVGHDRLF

SEQ ID NO: 11889 - protein, 9 aa, synthetic construct
GGVGHDTIY

SEQ ID NO: 11890 - protein, 9 aa, synthetic construct
GGKGADKMY

SEQ ID NO: 11891 - protein, 9 aa, synthetic construct
GGDGGDTLV

SEQ ID NO: 11892 - protein, 9 aa, synthetic construct
GGLGEDLLI

SEQ ID NO: 11893 - protein, 9 aa, synthetic construct
GGVGIDTMQ

SEQ ID NO: 11894 - protein, 9 aa, synthetic construct
GGQGDDVIY

SEQ ID NO: 11895 - protein, 9 aa, synthetic construct
GGDGGDTLY

SEQ ID NO: 11896 - protein, 9 aa, synthetic construct
GGAGIDYLY

SEQ ID NO: 11897 - protein, 9 aa, synthetic construct
GGAGKDAIF

SEQ ID NO: 11898 - protein, 9 aa, synthetic construct
GGLGEDRID

SEQ ID NO: 11899 - protein, 9 aa, synthetic construct
GGGGNDDIR

SEQ ID NO: 11900 - protein, 9 aa, synthetic construct
GGSGNDMLR

SEQ ID NO: 11901 - protein, 9 aa, synthetic construct
GGAGKDAIL

SEQ ID NO: 11902 - protein, 9 aa, synthetic construct
GGAGDDIFT

SEQ ID NO: 11903 - protein, 9 aa, synthetic construct
GGVGIDRLH

SEQ ID NO: 11904 - protein, 9 aa, synthetic construct
GGEGNDTVI

SEQ ID NO: 11905 - protein, 9 aa, synthetic construct
GGAGSDVID

SEQ ID NO: 11906 - protein, 9 aa, synthetic construct
GGLGEDRLT

SEQ ID NO: 11907 - protein, 9 aa, synthetic construct
GGSGTDVAT

SEQ ID NO: 11908 - protein, 9 aa, synthetic construct
GGSGNDMLD

SEQ ID NO: 11909 - protein, 9 aa, synthetic construct
GGEGSDLLQ

SEQ ID NO: 11910 - protein, 9 aa, synthetic construct
GGEGDDELL

SEQ ID NO: 11911 - protein, 9 aa, synthetic construct
GGAGSDVIS

SEQ ID NO: 11912 - protein, 9 aa, synthetic construct
GGAGDDIVT

SEQ ID NO: 11913 - protein, 9 aa, synthetic construct
GGHGNDILN

SEQ ID NO: 11914 - protein, 9 aa, synthetic construct
GGQGDDTMF

SEQ ID NO: 11915 - protein, 9 aa, synthetic construct
GGQGDDTML

SEQ ID NO: 11916 - protein, 9 aa, synthetic construct
GGQGDDTVF

SEQ ID NO: 11917 - protein, 9 aa, synthetic construct
GGGGNDSIY

SEQ ID NO: 11918 - protein, 9 aa, synthetic construct
GGSGNDNIR

SEQ ID NO: 11919 - protein, 9 aa, synthetic construct
GGAGDDIVS

SEQ ID NO: 11920 - protein, 9 aa, synthetic construct
GGLGDDYYI

SEQ ID NO: 11921 - protein, 9 aa, synthetic construct
GGFGNDRLN

SEQ ID NO: 11922 - protein, 9 aa, synthetic construct
GGSGTDTLL

SEQ ID NO: 11923 - protein, 9 aa, synthetic construct
GGSGNDMIG

SEQ ID NO: 11924 - protein, 9 aa, synthetic construct
GGHGNDAIT

SEQ ID NO: 11925 - protein, 9 aa, synthetic construct
GGGGNDDLW

SEQ ID NO: 11926 - protein, 9 aa, synthetic construct
GGDGLDFIN

SEQ ID NO: 11927 - protein, 9 aa, synthetic construct
GGNGDDLLT

SEQ ID NO: 11928 - protein, 9 aa, synthetic construct
GGSGTDTMT

SEQ ID NO: 11929 - protein, 9 aa, synthetic construct
GGSGTDVLD

SEQ ID NO: 11930 - protein, 9 aa, synthetic construct
GGMGNDTLR

SEQ ID NO: 11931 - protein, 9 aa, synthetic construct
GGAGDDIVF

SEQ ID NO: 11932 - protein, 9 aa, synthetic construct
GGEGSDLID

SEQ ID NO: 11933 - protein, 9 aa, synthetic construct
GGQGDDTYY

SEQ ID NO: 11934 - protein, 9 aa, synthetic construct
GGDGLDELR

SEQ ID NO: 11935 - protein, 9 aa, synthetic construct
GGHGNDRLS

SEQ ID NO: 11936 - protein, 9 aa, synthetic construct
GGQGDDRLL

SEQ ID NO: 11937 - protein, 9 aa, synthetic construct
GGAGDDKVT

SEQ ID NO: 11938 - protein, 9 aa, synthetic construct
GGQGDDLMG

SEQ ID NO: 11939 - protein, 9 aa, synthetic construct
GGVGDDSLI

SEQ ID NO: 11940 - protein, 9 aa, synthetic construct
GGQGMDALF

SEQ ID NO: 11941 - protein, 9 aa, synthetic construct
GGAGSDRIE

SEQ ID NO: 11942 - protein, 9 aa, synthetic construct
GGQGLDWMD

SEQ ID NO: 11943 - protein, 9 aa, synthetic construct
GGQGDDLLK

SEQ ID NO: 11944 - protein, 9 aa, synthetic construct
GGGGFDILV

SEQ ID NO: 11945 - protein, 9 aa, synthetic construct
GGVGDDSLV

SEQ ID NO: 11946 - protein, 9 aa, synthetic construct
GGEGDDEID

SEQ ID NO: 11947 - protein, 9 aa, synthetic construct
GGSGNDQLK

SEQ ID NO: 11948 - protein, 9 aa, synthetic construct
GGVGDDSLY

SEQ ID NO: 11949 - protein, 9 aa, synthetic construct
GGGGADVFY

SEQ ID NO: 11950 - protein, 9 aa, synthetic construct
GGDGKDTIT

SEQ ID NO: 11951 - protein, 9 aa, synthetic construct
GGLGDDVIN

SEQ ID NO: 11952 - protein, 9 aa, synthetic construct
GGQGLDRMF

SEQ ID NO: 11953 - protein, 9 aa, synthetic construct
GGHGNDTLN

SEQ ID NO: 11954 - protein, 9 aa, synthetic construct
GGKGADHFV

SEQ ID NO: 11955 - protein, 9 aa, synthetic construct
GGHGNDTLL

SEQ ID NO: 11956 - protein, 9 aa, synthetic construct
GGDGGDTYL

SEQ ID NO: 11957 - protein, 9 aa, synthetic construct
GGHGNDTLH

SEQ ID NO: 11958 - protein, 9 aa, synthetic construct
GGHGNDTLF

SEQ ID NO: 11959 - protein, 9 aa, synthetic construct
GGQGDDLVF

SEQ ID NO: 11960 - protein, 9 aa, synthetic construct
GGAGSDRLR

SEQ ID NO: 11961 - protein, 9 aa, synthetic construct
GGSGNDQLE

SEQ ID NO: 11962 - protein, 9 aa, synthetic construct
GGQGLDFAD

SEQ ID NO: 11963 - protein, 9 aa, synthetic construct
GGQGDDLLH

SEQ ID NO: 11964 - protein, 9 aa, synthetic construct
GGQGDDLLE

SEQ ID NO: 11965 - protein, 9 aa, synthetic construct
GGAGSDRFD

SEQ ID NO: 11966 - protein, 9 aa, synthetic construct
GGDGLDRLI

SEQ ID NO: 11967 - protein, 9 aa, synthetic construct
GGSGTDRLT

SEQ ID NO: 11968 - protein, 9 aa, synthetic construct
GGSGNDKVY

SEQ ID NO: 11969 - protein, 9 aa, synthetic construct
GGAGSDQIN

SEQ ID NO: 11970 - protein, 9 aa, synthetic construct
GGGGADVFH

SEQ ID NO: 11971 - protein, 9 aa, synthetic construct
GGAGDDLMN

SEQ ID NO: 11972 - protein, 9 aa, synthetic construct
GGGGDDALN

SEQ ID NO: 11973 - protein, 9 aa, synthetic construct
GGAGSDQLN

SEQ ID NO: 11974 - protein, 9 aa, synthetic construct
GGHGGDVIL

SEQ ID NO: 11975 - protein, 9 aa, synthetic construct
GGSGNDLFF

SEQ ID NO: 11976 - protein, 9 aa, synthetic construct
GGNGKDTLN

SEQ ID NO: 11977 - protein, 9 aa, synthetic construct
GGEGSDIIK

SEQ ID NO: 11978 - protein, 9 aa, synthetic construct
GGLGFDTLD

SEQ ID NO: 11979 - protein, 9 aa, synthetic construct
GGVGDDRLS

SEQ ID NO: 11980 - protein, 9 aa, synthetic construct
GGAGSDYLA

SEQ ID NO: 11981 - protein, 9 aa, synthetic construct
GGDGDDAIH

SEQ ID NO: 11982 - protein, 9 aa, synthetic construct
GGVGDDSID

SEQ ID NO: 11983 - protein, 9 aa, synthetic construct
GGHGNDTML

SEQ ID NO: 11984 - protein, 9 aa, synthetic construct
GGAGDDFVY

SEQ ID NO: 11985 - protein, 9 aa, synthetic construct
GGFGNDSFI

SEQ ID NO: 11986 - protein, 9 aa, synthetic construct
GGVGDDSLA

SEQ ID NO: 11987 - protein, 9 aa, synthetic construct
GGDGDDAII

SEQ ID NO: 11988 - protein, 9 aa, synthetic construct
GGAGSDRAS

SEQ ID NO: 11989 - protein, 9 aa, synthetic construct
GGQGMDTLL

SEQ ID NO: 11990 - protein, 9 aa, synthetic construct
GGEGADMLR

SEQ ID NO: 11991 - protein, 9 aa, synthetic construct
GGVGDDTVF

SEQ ID NO: 11992 - protein, 9 aa, synthetic construct
GGEGSDILS

SEQ ID NO: 11993 - protein, 9 aa, synthetic construct
GGGGNDALT

SEQ ID NO: 11994 - protein, 9 aa, synthetic construct
GGVGDDVMS

SEQ ID NO: 11995 - protein, 9 aa, synthetic construct
GGQGDDQLI

SEQ ID NO: 11996 - protein, 9 aa, synthetic construct
GGKGADLMV

SEQ ID NO: 11997 - protein, 9 aa, synthetic construct
GGKGADIIL

SEQ ID NO: 11998 - protein, 9 aa, synthetic construct
GGDGKDTLW

SEQ ID NO: 11999 - protein, 9 aa, synthetic construct
GGNGDDLLA

SEQ ID NO: 12000 - protein, 9 aa, synthetic construct
GGAGDDGLK

SEQ ID NO: 12001 - protein, 9 aa, synthetic construct
GGAGKDDLR

SEQ ID NO: 12002 - protein, 9 aa, synthetic construct
GGEGSDQLS

SEQ ID NO: 12003 - protein, 9 aa, synthetic construct
GGEGNDTLW

SEQ ID NO: 12004 - protein, 9 aa, synthetic construct
GGSGTDTAI

SEQ ID NO: 12005 - protein, 9 aa, synthetic construct
GGNGMDLIY

SEQ ID NO: 12006 - protein, 9 aa, synthetic construct
GGLGRDAIW

SEQ ID NO: 12007 - protein, 9 aa, synthetic construct
GGDGDDAIY

SEQ ID NO: 12008 - protein, 9 aa, synthetic construct
GGEGSDQLF

SEQ ID NO: 12009 - protein, 9 aa, synthetic construct
GGAGDDLAV

SEQ ID NO: 12010 - protein, 9 aa, synthetic construct
GGEGSDNMT

SEQ ID NO: 12011 - protein, 9 aa, synthetic construct
GGFGDDYIL

SEQ ID NO: 12012 - protein, 9 aa, synthetic construct
GGVGDDYLV

SEQ ID NO: 12013 - protein, 9 aa, synthetic construct
GGEGNDDLY

SEQ ID NO: 12014 - protein, 9 aa, synthetic construct
GGAGDDLAD

SEQ ID NO: 12015 - protein, 9 aa, synthetic construct
GGEGDDEIH

SEQ ID NO: 12016 - protein, 9 aa, synthetic construct
GGGGADVLQ

SEQ ID NO: 12017 - protein, 9 aa, synthetic construct
GGQGDDRLE

SEQ ID NO: 12018 - protein, 9 aa, synthetic construct
GGAGIDVMI

SEQ ID NO: 12019 - protein, 9 aa, synthetic construct
GGDGDDMLI

SEQ ID NO: 12020 - protein, 9 aa, synthetic construct
GGVGDDVLR

SEQ ID NO: 12021 - protein, 9 aa, synthetic construct
GGVGNDAIV

SEQ ID NO: 12022 - protein, 9 aa, synthetic construct
GGEGSDILI

SEQ ID NO: 12023 - protein, 9 aa, synthetic construct
GGSGNDLIS

SEQ ID NO: 12024 - protein, 9 aa, synthetic construct
GGAGSDRMY

SEQ ID NO: 12025 - protein, 9 aa, synthetic construct
GGLGDDVIV

SEQ ID NO: 12026 - protein, 9 aa, synthetic construct
GGVGNDALV

SEQ ID NO: 12027 - protein, 9 aa, synthetic construct
GGAGIDVLL

SEQ ID NO: 12028 - protein, 9 aa, synthetic construct
GGQGKDTIF

SEQ ID NO: 12029 - protein, 9 aa, synthetic construct
GGVGDDTYT

SEQ ID NO: 12030 - protein, 9 aa, synthetic construct
GGGGRDQLY

SEQ ID NO: 12031 - protein, 9 aa, synthetic construct
GGGGDDAIG

SEQ ID NO: 12032 - protein, 9 aa, synthetic construct
GGLGFDLLE

SEQ ID NO: 12033 - protein, 9 aa, synthetic construct
GGEGADVFA

SEQ ID NO: 12034 - protein, 9 aa, synthetic construct
GGGGNDSIN

SEQ ID NO: 12035 - protein, 9 aa, synthetic construct
GGGGADVIL

SEQ ID NO: 12036 - protein, 9 aa, synthetic construct
GGAGSDWLK

SEQ ID NO: 12037 - protein, 9 aa, synthetic construct
GGVGDDVII

SEQ ID NO: 12038 - protein, 9 aa, synthetic construct
GGKGADHLY

SEQ ID NO: 12039 - protein, 9 aa, synthetic construct
GGAGDDLFY

SEQ ID NO: 12040 - protein, 9 aa, synthetic construct
GGDGFDTYH

SEQ ID NO: 12041 - protein, 9 aa, synthetic construct
GGVGDDVLD

SEQ ID NO: 12042 - protein, 9 aa, synthetic construct
GGGGADVLA

SEQ ID NO: 12043 - protein, 9 aa, synthetic construct
GGAGIDVLY

SEQ ID NO: 12044 - protein, 9 aa, synthetic construct
GGNGDDLIR

SEQ ID NO: 12045 - protein, 9 aa, synthetic construct
GGVGNDRIE

SEQ ID NO: 12046 - protein, 9 aa, synthetic construct
GGSGVDVIY

SEQ ID NO: 12047 - protein, 9 aa, synthetic construct
GGQGADRLE

SEQ ID NO: 12048 - protein, 9 aa, synthetic construct
GGTGTDMLI

SEQ ID NO: 12049 - protein, 9 aa, synthetic construct
GGAGDDTMN

SEQ ID NO: 12050 - protein, 9 aa, synthetic construct
GGRGADQMT

SEQ ID NO: 12051 - protein, 9 aa, synthetic construct
GGTGTDLLN

SEQ ID NO: 12052 - protein, 9 aa, synthetic construct
GGGGNDTFD

SEQ ID NO: 12053 - protein, 9 aa, synthetic construct
GGGGADQLT

SEQ ID NO: 12054 - protein, 9 aa, synthetic construct
GGGGDDIIG

SEQ ID NO: 12055 - protein, 9 aa, synthetic construct
GGAGRDTML

SEQ ID NO: 12056 - protein, 9 aa, synthetic construct
GGDGADXID

SEQ ID NO: 12057 - protein, 9 aa, synthetic construct
GGLGSDSYG

SEQ ID NO: 12058 - protein, 9 aa, synthetic construct
GGAGTDTVT

SEQ ID NO: 12059 - protein, 9 aa, synthetic construct
GGRGADNLD

SEQ ID NO: 12060 - protein, 9 aa, synthetic construct
GGSGYDRVY

SEQ ID NO: 12061 - protein, 9 aa, synthetic construct
GGRGADRFV

SEQ ID NO: 12062 - protein, 9 aa, synthetic construct
GGAGDDAMF

SEQ ID NO: 12063 - protein, 9 aa, synthetic construct
GGRGADMLN

SEQ ID NO: 12064 - protein, 9 aa, synthetic construct
GGLGDDIIE

SEQ ID NO: 12065 - protein, 9 aa, synthetic construct
GGAGNDAIV

SEQ ID NO: 12066 - protein, 9 aa, synthetic construct
GGAGTDTVD

SEQ ID NO: 12067 - protein, 9 aa, synthetic construct
GGAGTDTMY

SEQ ID NO: 12068 - protein, 9 aa, synthetic construct
GGAGIDRMT

SEQ ID NO: 12069 - protein, 9 aa, synthetic construct
GGLGVDTAV

SEQ ID NO: 12070 - protein, 9 aa, synthetic construct
GGTGTDQLA

SEQ ID NO: 12071 - protein, 9 aa, synthetic construct
GGSGNDEIE

SEQ ID NO: 12072 - protein, 9 aa, synthetic construct
GGEGGDTID

SEQ ID NO: 12073 - protein, 9 aa, synthetic construct
GGLGQDSLT

SEQ ID NO: 12074 - protein, 9 aa, synthetic construct
GGSGYDTAS

SEQ ID NO: 12075 - protein, 9 aa, synthetic construct
GGSGTDILN

SEQ ID NO: 12076 - protein, 9 aa, synthetic construct
GGDGIDTIY

SEQ ID NO: 12077 - protein, 9 aa, synthetic construct
GGRGADTFA

SEQ ID NO: 12078 - protein, 9 aa, synthetic construct
GGSGYDTLY

SEQ ID NO: 12079 - protein, 9 aa, synthetic construct
GGPGRDRLF

SEQ ID NO: 12080 - protein, 9 aa, synthetic construct
GGSGNDDLF

SEQ ID NO: 12081 - protein, 9 aa, synthetic construct
GGPGRDRLT

SEQ ID NO: 12082 - protein, 9 aa, synthetic construct
GGAGDDTYE

SEQ ID NO: 12083 - protein, 9 aa, synthetic construct
GGSGNDDLL

SEQ ID NO: 12084 - protein, 9 aa, synthetic construct
GGSGNDDLN

SEQ ID NO: 12085 - protein, 9 aa, synthetic construct
GGSGNDDLQ

SEQ ID NO: 12086 - protein, 9 aa, synthetic construct
GGSGYDTLN

SEQ ID NO: 12087 - protein, 9 aa, synthetic construct
GGSGNDSMG

SEQ ID NO: 12088 - protein, 9 aa, synthetic construct
GGLGTDTLS

SEQ ID NO: 12089 - protein, 9 aa, synthetic construct
GGVGQDTLD

SEQ ID NO: 12090 - protein, 9 aa, synthetic construct
GGEGADLLY

SEQ ID NO: 12091 - protein, 9 aa, synthetic construct
GGRGADRMA

SEQ ID NO: 12092 - protein, 9 aa, synthetic construct
GGIGVDSMV

SEQ ID NO: 12093 - protein, 9 aa, synthetic construct
GGAGDDTVG

SEQ ID NO: 12094 - protein, 9 aa, synthetic construct
GGLGIDSLT

SEQ ID NO: 12095 - protein, 9 aa, synthetic construct
GGAGDDALE

SEQ ID NO: 12096 - protein, 9 aa, synthetic construct
GGGGRDTII

SEQ ID NO: 12097 - protein, 9 aa, synthetic construct
GGVGQDTLI

SEQ ID NO: 12098 - protein, 9 aa, synthetic construct
GGRGADRLE

SEQ ID NO: 12099 - protein, 9 aa, synthetic construct
GGAGDDTMV

SEQ ID NO: 12100 - protein, 9 aa, synthetic construct
GGPGRDTLI

SEQ ID NO: 12101 - protein, 9 aa, synthetic construct
GGDGGDWID

SEQ ID NO: 12102 - protein, 9 aa, synthetic construct
GGGGNDRYY

SEQ ID NO: 12103 - protein, 9 aa, synthetic construct
GGDGIDTLY

SEQ ID NO: 12104 - protein, 9 aa, synthetic construct
GGAGDDCLV

SEQ ID NO: 12105 - protein, 9 aa, synthetic construct
GGSGSDWLE

SEQ ID NO: 12106 - protein, 9 aa, synthetic construct
GGPGSDNFY

SEQ ID NO: 12107 - protein, 9 aa, synthetic construct
GGDGIDTVE

SEQ ID NO: 12108 - protein, 9 aa, synthetic construct
GGGGHDRLV

SEQ ID NO: 12109 - protein, 9 aa, synthetic construct
GGDGADYIK

SEQ ID NO: 12110 - protein, 9 aa, synthetic construct
GGLGSDRLF

SEQ ID NO: 12111 - protein, 9 aa, synthetic construct
GGAGRDVIT

SEQ ID NO: 12112 - protein, 9 aa, synthetic construct
GGGGRDTFR

SEQ ID NO: 12113 - protein, 9 aa, synthetic construct
GGPGSDQLS

SEQ ID NO: 12114 - protein, 9 aa, synthetic construct
GGKGADRMI

SEQ ID NO: 12115 - protein, 9 aa, synthetic construct
GGAGRDVIY

SEQ ID NO: 12116 - protein, 9 aa, synthetic construct
GGMGNDHMT

SEQ ID NO: 12117 - protein, 9 aa, synthetic construct
GGAGTDTML

SEQ ID NO: 12118 - protein, 9 aa, synthetic construct
GGSGNDELR

SEQ ID NO: 12119 - protein, 9 aa, synthetic construct
GGVGNDWLA

SEQ ID NO: 12120 - protein, 9 aa, synthetic construct
GGRGADAFV

SEQ ID NO: 12121 - protein, 9 aa, synthetic construct
GGRGADAAD

SEQ ID NO: 12122 - protein, 9 aa, synthetic construct
GGSGYDLLT

SEQ ID NO: 12123 - protein, 9 aa, synthetic construct
GGTGTDTVD

SEQ ID NO: 12124 - protein, 9 aa, synthetic construct
GGAGDDDIE

SEQ ID NO: 12125 - protein, 9 aa, synthetic construct
GGAGKDILV

SEQ ID NO: 12126 - protein, 9 aa, synthetic construct
GGTGTDTYS

SEQ ID NO: 12127 - protein, 9 aa, synthetic construct
GGNGDDTVT

SEQ ID NO: 12128 - protein, 9 aa, synthetic construct
GGEGSDTVT

SEQ ID NO: 12129 - protein, 9 aa, synthetic construct
GGLGDDIYF

SEQ ID NO: 12130 - protein, 9 aa, synthetic construct
GGTGTDTLS

SEQ ID NO: 12131 - protein, 9 aa, synthetic construct
GGTGTDTLH

SEQ ID NO: 12132 - protein, 9 aa, synthetic construct
GGAGTDTIV

SEQ ID NO: 12133 - protein, 9 aa, synthetic construct
GGSGNDEIF

SEQ ID NO: 12134 - protein, 9 aa, synthetic construct
GGAGTDTMI

SEQ ID NO: 12135 - protein, 9 aa, synthetic construct
GGLGVDTAN

SEQ ID NO: 12136 - protein, 9 aa, synthetic construct
GGRGADKMF

SEQ ID NO: 12137 - protein, 9 aa, synthetic construct
GGGGRDTIA

SEQ ID NO: 12138 - protein, 9 aa, synthetic construct
GGEGNDFIN

SEQ ID NO: 12139 - protein, 9 aa, synthetic construct
GGLGIDKLI

SEQ ID NO: 12140 - protein, 9 aa, synthetic construct
GGLGDDILL

SEQ ID NO: 12141 - protein, 9 aa, synthetic construct
GGLGTDTMI

SEQ ID NO: 12142 - protein, 9 aa, synthetic construct
GGTGTDTAD

SEQ ID NO: 12143 - protein, 9 aa, synthetic construct
GGRGADILI

SEQ ID NO: 12144 - protein, 9 aa, synthetic construct
GGEGNDFIL

SEQ ID NO: 12145 - protein, 9 aa, synthetic construct
GGIGADLLY

SEQ ID NO: 12146 - protein, 9 aa, synthetic construct
GGTGTDTAT

SEQ ID NO: 12147 - protein, 9 aa, synthetic construct
GGEGNDTFI

SEQ ID NO: 12148 - protein, 9 aa, synthetic construct
GGSGYDQLS

SEQ ID NO: 12149 - protein, 9 aa, synthetic construct
GGAGDDTFY

SEQ ID NO: 12150 - protein, 9 aa, synthetic construct
GGPGSDILN

SEQ ID NO: 12151 - protein, 9 aa, synthetic construct
GGAGTDTLF

SEQ ID NO: 12152 - protein, 9 aa, synthetic construct
GGAGTDTLE

SEQ ID NO: 12153 - protein, 9 aa, synthetic construct
GGLGDDIMR

SEQ ID NO: 12154 - protein, 9 aa, synthetic construct
GGGGADRFL

SEQ ID NO: 12155 - protein, 9 aa, synthetic construct
GGGGRDTFS

SEQ ID NO: 12156 - protein, 9 aa, synthetic construct
GGDGIDTIS

SEQ ID NO: 12157 - protein, 9 aa, synthetic construct
GGDGSDTMS

SEQ ID NO: 12158 - protein, 9 aa, synthetic construct
GGRGADTFL

SEQ ID NO: 12159 - protein, 9 aa, synthetic construct
GGEGRDVLS

SEQ ID NO: 12160 - protein, 9 aa, synthetic construct
GGTGADALY

SEQ ID NO: 12161 - protein, 9 aa, synthetic construct
GGLGDDELQ

SEQ ID NO: 12162 - protein, 9 aa, synthetic construct
GGTGSDTAA

SEQ ID NO: 12163 - protein, 9 aa, synthetic construct
GGDGIDTAA

SEQ ID NO: 12164 - protein, 9 aa, synthetic construct
GGAGRDSAV

SEQ ID NO: 12165 - protein, 9 aa, synthetic construct
GGSGSDVFY

SEQ ID NO: 12166 - protein, 9 aa, synthetic construct
GGHGADTLT

SEQ ID NO: 12167 - protein, 9 aa, synthetic construct
GGNGNDIFI

SEQ ID NO: 12168 - protein, 9 aa, synthetic construct
GGAGRDSFQ

SEQ ID NO: 12169 - protein, 9 aa, synthetic construct
GGRGDDELI

SEQ ID NO: 12170 - protein, 9 aa, synthetic construct
GGTGSDTAV

SEQ ID NO: 12171 - protein, 9 aa, synthetic construct
GGTGSDTFK

SEQ ID NO: 12172 - protein, 9 aa, synthetic construct
GGGGDDIVH

SEQ ID NO: 12173 - protein, 9 aa, synthetic construct
GGLGIDTVV

SEQ ID NO: 12174 - protein, 9 aa, synthetic construct
GGPGQDTLT

SEQ ID NO: 12175 - protein, 9 aa, synthetic construct
GGAGRDSIL

SEQ ID NO: 12176 - protein, 9 aa, synthetic construct
GGTGSDTFT

SEQ ID NO: 12177 - protein, 9 aa, synthetic construct
GGKGHDTLD

SEQ ID NO: 12178 - protein, 9 aa, synthetic construct
GGAGRDSIT

SEQ ID NO: 12179 - protein, 9 aa, synthetic construct
GGDGDDELW

SEQ ID NO: 12180 - protein, 9 aa, synthetic construct
GGTGSDTIH

SEQ ID NO: 12181 - protein, 9 aa, synthetic construct
GGAGRDSLD

SEQ ID NO: 12182 - protein, 9 aa, synthetic construct
GGDGDDLYY

SEQ ID NO: 12183 - protein, 9 aa, synthetic construct
GGSGNDSVS

SEQ ID NO: 12184 - protein, 9 aa, synthetic construct
GGEGDDHML

SEQ ID NO: 12185 - protein, 9 aa, synthetic construct
GGLGDDELK

SEQ ID NO: 12186 - protein, 9 aa, synthetic construct
GGDGNDALL

SEQ ID NO: 12187 - protein, 9 aa, synthetic construct
GGGGADNLS

SEQ ID NO: 12188 - protein, 9 aa, synthetic construct
GGAGNDAYH

SEQ ID NO: 12189 - protein, 9 aa, synthetic construct
GGTGADAMS

SEQ ID NO: 12190 - protein, 9 aa, synthetic construct
GGTGADAMN

SEQ ID NO: 12191 - protein, 9 aa, synthetic construct
GGAGDDVMG

SEQ ID NO: 12192 - protein, 9 aa, synthetic construct
GGKGHDTLL

SEQ ID NO: 12193 - protein, 9 aa, synthetic construct
GGSGNDAID

SEQ ID NO: 12194 - protein, 9 aa, synthetic construct
GGTGSDRLE

SEQ ID NO: 12195 - protein, 9 aa, synthetic construct
GGTGSDRLI

SEQ ID NO: 12196 - protein, 9 aa, synthetic construct
GGGGEDTLY

SEQ ID NO: 12197 - protein, 9 aa, synthetic construct
GGDGSDTIV

SEQ ID NO: 12198 - protein, 9 aa, synthetic construct
GGTGSDRLY

SEQ ID NO: 12199 - protein, 9 aa, synthetic construct
GGRGDDGLH

SEQ ID NO: 12200 - protein, 9 aa, synthetic construct
GGTGADAMD

SEQ ID NO: 12201 - protein, 9 aa, synthetic construct
GGLGKDFLS

SEQ ID NO: 12202 - protein, 9 aa, synthetic construct
GGLGQDSLF

SEQ ID NO: 12203 - protein, 9 aa, synthetic construct
GGKGDDWLS

SEQ ID NO: 12204 - protein, 9 aa, synthetic construct
GGVGRDVLI

SEQ ID NO: 12205 - protein, 9 aa, synthetic construct
GGSGNDALA

SEQ ID NO: 12206 - protein, 9 aa, synthetic construct
GGNGNDIFR

SEQ ID NO: 12207 - protein, 9 aa, synthetic construct
GGGGADNLN

SEQ ID NO: 12208 - protein, 9 aa, synthetic construct
GGLGDDELD

SEQ ID NO: 12209 - protein, 9 aa, synthetic construct
GGLGDDELF

SEQ ID NO: 12210 - protein, 9 aa, synthetic construct
GGRGDDFLF

SEQ ID NO: 12211 - protein, 9 aa, synthetic construct
GGAGLDTMT

SEQ ID NO: 12212 - protein, 9 aa, synthetic construct
GGAGRDSLR

SEQ ID NO: 12213 - protein, 9 aa, synthetic construct
GGTGSDYLS

SEQ ID NO: 12214 - protein, 9 aa, synthetic construct
GGAGDDAID

SEQ ID NO: 12215 - protein, 9 aa, synthetic construct
GGTGSDVLR

SEQ ID NO: 12216 - protein, 9 aa, synthetic construct
GGGGRDTLA

SEQ ID NO: 12217 - protein, 9 aa, synthetic construct
GGNGIDLLF

SEQ ID NO: 12218 - protein, 9 aa, synthetic construct
GGEGRDYLF

SEQ ID NO: 12219 - protein, 9 aa, synthetic construct
GGAGIDRLE

SEQ ID NO: 12220 - protein, 9 aa, synthetic construct
GGNGNDHLL

SEQ ID NO: 12221 - protein, 9 aa, synthetic construct
GGDGQDLAM

SEQ ID NO: 12222 - protein, 9 aa, synthetic construct
GGLGDDGLT

SEQ ID NO: 12223 - protein, 9 aa, synthetic construct
GGAGRDTIA

SEQ ID NO: 12224 - protein, 9 aa, synthetic construct
GGAGTDVLV

SEQ ID NO: 12225 - protein, 9 aa, synthetic construct
GGEGADRLT

SEQ ID NO: 12226 - protein, 9 aa, synthetic construct
GGSGNDDIE

SEQ ID NO: 12227 - protein, 9 aa, synthetic construct
GGHGADTVL

SEQ ID NO: 12228 - protein, 9 aa, synthetic construct
GGIGADRMA

SEQ ID NO: 12229 - protein, 9 aa, synthetic construct
GGIGADRLY

SEQ ID NO: 12230 - protein, 9 aa, synthetic construct
GGSGSDVLF

SEQ ID NO: 12231 - protein, 9 aa, synthetic construct
GGSGNDDIR

SEQ ID NO: 12232 - protein, 9 aa, synthetic construct
GGGGADQLR

SEQ ID NO: 12233 - protein, 9 aa, synthetic construct
GGAGRDTII

SEQ ID NO: 12234 - protein, 9 aa, synthetic construct
GGAGTDVIR

SEQ ID NO: 12235 - protein, 9 aa, synthetic construct
GGRGADTII

SEQ ID NO: 12236 - protein, 9 aa, synthetic construct
GGTGSDYLN

SEQ ID NO: 12237 - protein, 9 aa, synthetic construct
GGLGRDQLF

SEQ ID NO: 12238 - protein, 9 aa, synthetic construct
GGAGDDAIL

SEQ ID NO: 12239 - protein, 9 aa, synthetic construct
GGAGDDVFL

SEQ ID NO: 12240 - protein, 9 aa, synthetic construct
GGAGIDHLY

SEQ ID NO: 12241 - protein, 9 aa, synthetic construct
GGTGSDVID

SEQ ID NO: 12242 - protein, 9 aa, synthetic construct
GGAGNDAMH

SEQ ID NO: 12243 - protein, 9 aa, synthetic construct
GGSGNDAMT

SEQ ID NO: 12244 - protein, 9 aa, synthetic construct
GGAGTDYIA

SEQ ID NO: 12245 - protein, 9 aa, synthetic construct
GGTGSDTMN

SEQ ID NO: 12246 - protein, 9 aa, synthetic construct
GGLGDDFLF

SEQ ID NO: 12247 - protein, 9 aa, synthetic construct
GGSGNDSVG

SEQ ID NO: 12248 - protein, 9 aa, synthetic construct
GGGGDDIMI

SEQ ID NO: 12249 - protein, 9 aa, synthetic construct
GGHGADVIN

SEQ ID NO: 12250 - protein, 9 aa, synthetic construct
GGTGSDTMY

SEQ ID NO: 12251 - protein, 9 aa, synthetic construct
GGAGNDAMV

SEQ ID NO: 12252 - protein, 9 aa, synthetic construct
GGGGNDIII

SEQ ID NO: 12253 - protein, 9 aa, synthetic construct
GGGGRDTLK

SEQ ID NO: 12254 - protein, 9 aa, synthetic construct
GGEGNDVVD

SEQ ID NO: 12255 - protein, 9 aa, synthetic construct
GGAGCDILN

SEQ ID NO: 12256 - protein, 9 aa, synthetic construct
GGLGDDFLV

SEQ ID NO: 12257 - protein, 9 aa, synthetic construct
GGPGRDILE

SEQ ID NO: 12258 - protein, 9 aa, synthetic construct
GGGGLDKIY

SEQ ID NO: 12259 - protein, 9 aa, synthetic construct
GGFGNDTIT

SEQ ID NO: 12260 - protein, 9 aa, synthetic construct
GGAGDDVFT

SEQ ID NO: 12261 - protein, 9 aa, synthetic construct
GGRGADVLN

SEQ ID NO: 12262 - protein, 9 aa, synthetic construct
GGAGNDAML

SEQ ID NO: 12263 - protein, 9 aa, synthetic construct
GGAGRDTAV

SEQ ID NO: 12264 - protein, 9 aa, synthetic construct
GGRGADVLE

SEQ ID NO: 12265 - protein, 9 aa, synthetic construct
GGAGDDVFQ

SEQ ID NO: 12266 - protein, 9 aa, synthetic construct
GGNGDDIMF

SEQ ID NO: 12267 - protein, 9 aa, synthetic construct
GGKGHDSID

SEQ ID NO: 12268 - protein, 9 aa, synthetic construct
GGAGIDSIF

SEQ ID NO: 12269 - protein, 9 aa, synthetic construct
GGNGDDTVE

SEQ ID NO: 12270 - protein, 9 aa, synthetic construct
GGAGSDFAN

SEQ ID NO: 12271 - protein, 9 aa, synthetic construct
GGLGDDMVF

SEQ ID NO: 12272 - protein, 9 aa, synthetic construct
GGLGTDVLN

SEQ ID NO: 12273 - protein, 9 aa, synthetic construct
GGDGKDFVF

SEQ ID NO: 12274 - protein, 9 aa, synthetic construct
GGLGHDILV

SEQ ID NO: 12275 - protein, 9 aa, synthetic construct
GGDGFDAAS

SEQ ID NO: 12276 - protein, 9 aa, synthetic construct
GGKGADALH

SEQ ID NO: 12277 - protein, 9 aa, synthetic construct
GGTGYDTLY

SEQ ID NO: 12278 - protein, 9 aa, synthetic construct
GGVGNDSMV

SEQ ID NO: 12279 - protein, 9 aa, synthetic construct
GGLGDDNLR

SEQ ID NO: 12280 - protein, 9 aa, synthetic construct
GGAGDDRLG

SEQ ID NO: 12281 - protein, 9 aa, synthetic construct
GGDGSDWLD

SEQ ID NO: 12282 - protein, 9 aa, synthetic construct
GGVGNDSLV

SEQ ID NO: 12283 - protein, 9 aa, synthetic construct
GGLGDDNLV

SEQ ID NO: 12284 - protein, 9 aa, synthetic construct
GGQGRDTLD

SEQ ID NO: 12285 - protein, 9 aa, synthetic construct
GGNGKDFLY

SEQ ID NO: 12286 - protein, 9 aa, synthetic construct
GGAGDDEID

SEQ ID NO: 12287 - protein, 9 aa, synthetic construct
GGAGSDFLH

SEQ ID NO: 12288 - protein, 9 aa, synthetic construct
GGSGNDGLY

SEQ ID NO: 12289 - protein, 9 aa, synthetic construct
GGVGADDLY

SEQ ID NO: 12290 - protein, 9 aa, synthetic construct
GGGGNDTAF

SEQ ID NO: 12291 - protein, 9 aa, synthetic construct
GGEGSDTIA

SEQ ID NO: 12292 - protein, 9 aa, synthetic construct
GGLGQDTLK

SEQ ID NO: 12293 - protein, 9 aa, synthetic construct
GGNGKDFYI

SEQ ID NO: 12294 - protein, 9 aa, synthetic construct
GGTGYDRIY

SEQ ID NO: 12295 - protein, 9 aa, synthetic construct
GGHGDDTLD

SEQ ID NO: 12296 - protein, 9 aa, synthetic construct
GGQGSDDAA

SEQ ID NO: 12297 - protein, 9 aa, synthetic construct
GGGGGDTLQ

SEQ ID NO: 12298 - protein, 9 aa, synthetic construct
GGQGSDLLL

SEQ ID NO: 12299 - protein, 9 aa, synthetic construct
GGGGADSIL

SEQ ID NO: 12300 - protein, 9 aa, synthetic construct
GGEGSDTIL

SEQ ID NO: 12301 - protein, 9 aa, synthetic construct
GGEGDDFVN

SEQ ID NO: 12302 - protein, 9 aa, synthetic construct
GGEGSDTII

SEQ ID NO: 12303 - protein, 9 aa, synthetic construct
GGPGYDILI

SEQ ID NO: 12304 - protein, 9 aa, synthetic construct
GGIGADALL

SEQ ID NO: 12305 - protein, 9 aa, synthetic construct
GGAGDDRVF

SEQ ID NO: 12306 - protein, 9 aa, synthetic construct
GGAGSDEIR

SEQ ID NO: 12307 - protein, 9 aa, synthetic construct
GGAGDDRMY

SEQ ID NO: 12308 - protein, 9 aa, synthetic construct
GGQGSDILS

SEQ ID NO: 12309 - protein, 9 aa, synthetic construct
GGQGSDILI

SEQ ID NO: 12310 - protein, 9 aa, synthetic construct
GGQGSDIFV

SEQ ID NO: 12311 - protein, 9 aa, synthetic construct
GGLGDDMLN

SEQ ID NO: 12312 - protein, 9 aa, synthetic construct
GGHGDDTID

SEQ ID NO: 12313 - protein, 9 aa, synthetic construct
GGAGSDELI

SEQ ID NO: 12314 - protein, 9 aa, synthetic construct
GGQGSDFYY

SEQ ID NO: 12315 - protein, 9 aa, synthetic construct
GGAGDDRMS

SEQ ID NO: 12316 - protein, 9 aa, synthetic construct
GGAGDDDVN

SEQ ID NO: 12317 - protein, 9 aa, synthetic construct
GGAGDDRMQ

SEQ ID NO: 12318 - protein, 9 aa, synthetic construct
GGNGNDFIR

SEQ ID NO: 12319 - protein, 9 aa, synthetic construct
GGAGDDRMN

SEQ ID NO: 12320 - protein, 9 aa, synthetic construct
GGSGNDSFI

SEQ ID NO: 12321 - protein, 9 aa, synthetic construct
GGDGKDILA

SEQ ID NO: 12322 - protein, 9 aa, synthetic construct
GGDGDDVAS

SEQ ID NO: 12323 - protein, 9 aa, synthetic construct
GGAGSDDVR

SEQ ID NO: 12324 - protein, 9 aa, synthetic construct
GGVGADLLD

SEQ ID NO: 12325 - protein, 9 aa, synthetic construct
GGDGGDTFL

SEQ ID NO: 12326 - protein, 9 aa, synthetic construct
GGSGNDHLD

SEQ ID NO: 12327 - protein, 9 aa, synthetic construct
GGAGSDIIA

SEQ ID NO: 12328 - protein, 9 aa, synthetic construct
GGVGNDRMW

SEQ ID NO: 12329 - protein, 9 aa, synthetic construct
GGLGDDRIG

SEQ ID NO: 12330 - protein, 9 aa, synthetic construct
GGLGGDVLT

SEQ ID NO: 12331 - protein, 9 aa, synthetic construct
GGNGDDTLG

SEQ ID NO: 12332 - protein, 9 aa, synthetic construct
GGQGQDRLI

SEQ ID NO: 12333 - protein, 9 aa, synthetic construct
GGSGNDRMK

SEQ ID NO: 12334 - protein, 9 aa, synthetic construct
GGLGDDRIY

SEQ ID NO: 12335 - protein, 9 aa, synthetic construct
GGEGNDTIM

SEQ ID NO: 12336 - protein, 9 aa, synthetic construct
GGSGNDRMF

SEQ ID NO: 12337 - protein, 9 aa, synthetic construct
GGMGRDWLA

SEQ ID NO: 12338 - protein, 9 aa, synthetic construct
GGAGTDLLF

SEQ ID NO: 12339 - protein, 9 aa, synthetic construct
GGDGDDMLT

SEQ ID NO: 12340 - protein, 9 aa, synthetic construct
GGHGDDTLS

SEQ ID NO: 12341 - protein, 9 aa, synthetic construct
GGLGGDVLD

SEQ ID NO: 12342 - protein, 9 aa, synthetic construct
GGQGQDILN

SEQ ID NO: 12343 - protein, 9 aa, synthetic construct
GGAGSDILL

SEQ ID NO: 12344 - protein, 9 aa, synthetic construct
GGQGADQLY

SEQ ID NO: 12345 - protein, 9 aa, synthetic construct
GGEGDDDLR

SEQ ID NO: 12346 - protein, 9 aa, synthetic construct
GGQGQDFIA

SEQ ID NO: 12347 - protein, 9 aa, synthetic construct
GGQGQDELI

SEQ ID NO: 12348 - protein, 9 aa, synthetic construct
GGVGADLMI

SEQ ID NO: 12349 - protein, 9 aa, synthetic construct
GGLGDDRFV

SEQ ID NO: 12350 - protein, 9 aa, synthetic construct
GGAGTDLMY

SEQ ID NO: 12351 - protein, 9 aa, synthetic construct
GGQGADLLN

SEQ ID NO: 12352 - protein, 9 aa, synthetic construct
GGAGKDHMS

SEQ ID NO: 12353 - protein, 9 aa, synthetic construct
GGGGIDRFY

SEQ ID NO: 12354 - protein, 9 aa, synthetic construct
GGTGDDHLS

SEQ ID NO: 12355 - protein, 9 aa, synthetic construct
GGVGNDSLA

SEQ ID NO: 12356 - protein, 9 aa, synthetic construct
GGEGSDTFI

SEQ ID NO: 12357 - protein, 9 aa, synthetic construct
GGAGIDTAF

SEQ ID NO: 12358 - protein, 9 aa, synthetic construct
GGAGSDHID

SEQ ID NO: 12359 - protein, 9 aa, synthetic construct
GGLGDDQLN

SEQ ID NO: 12360 - protein, 9 aa, synthetic construct
GGDGLDVLY

SEQ ID NO: 12361 - protein, 9 aa, synthetic construct
GGQGADIMS

SEQ ID NO: 12362 - protein, 9 aa, synthetic construct
GGVGNDSII

SEQ ID NO: 12363 - protein, 9 aa, synthetic construct
GGQGADIMY

SEQ ID NO: 12364 - protein, 9 aa, synthetic construct
GGDGLDVLT

SEQ ID NO: 12365 - protein, 9 aa, synthetic construct
GGAGMDTVS

SEQ ID NO: 12366 - protein, 9 aa, synthetic construct
GGEGDDFLV

SEQ ID NO: 12367 - protein, 9 aa, synthetic construct
GGAGSDHLV

SEQ ID NO: 12368 - protein, 9 aa, synthetic construct
GGGGADTFN

SEQ ID NO: 12369 - protein, 9 aa, synthetic construct
GGDGLDVLL

SEQ ID NO: 12370 - protein, 9 aa, synthetic construct
GGDGSDYIE

SEQ ID NO: 12371 - protein, 9 aa, synthetic construct
GGNGKDKLF

SEQ ID NO: 12372 - protein, 9 aa, synthetic construct
GGNGNDELQ

SEQ ID NO: 12373 - protein, 9 aa, synthetic construct
GGDGDDWLN

SEQ ID NO: 12374 - protein, 9 aa, synthetic construct
GGQGADLLA

SEQ ID NO: 12375 - protein, 9 aa, synthetic construct
GGVGADKLD

SEQ ID NO: 12376 - protein, 9 aa, synthetic construct
GGAGDDDMS

SEQ ID NO: 12377 - protein, 9 aa, synthetic construct
GGGGADSIE

SEQ ID NO: 12378 - protein, 9 aa, synthetic construct
GGHGDDNIL

SEQ ID NO: 12379 - protein, 9 aa, synthetic construct
GGTGVDIMN

SEQ ID NO: 12380 - protein, 9 aa, synthetic construct
GGLGHDVLL

SEQ ID NO: 12381 - protein, 9 aa, synthetic construct
GGPGSDTYY

SEQ ID NO: 12382 - protein, 9 aa, synthetic construct
GGEGADVFS

SEQ ID NO: 12383 - protein, 9 aa, synthetic construct
GGQGVDNLL

SEQ ID NO: 12384 - protein, 9 aa, synthetic construct
GGAGRDWLI

SEQ ID NO: 12385 - protein, 9 aa, synthetic construct
GGAGDDDIT

SEQ ID NO: 12386 - protein, 9 aa, synthetic construct
GGVGNDVLH

SEQ ID NO: 12387 - protein, 9 aa, synthetic construct
GGEGNDTFR

SEQ ID NO: 12388 - protein, 9 aa, synthetic construct
GGKGHDRIL

SEQ ID NO: 12389 - protein, 9 aa, synthetic construct
GGLGHDTYV

SEQ ID NO: 12390 - protein, 9 aa, synthetic construct
GGSGNDSIN

SEQ ID NO: 12391 - protein, 9 aa, synthetic construct
GGVGNDVLA

SEQ ID NO: 12392 - protein, 9 aa, synthetic construct
GGAGDDSMA

SEQ ID NO: 12393 - protein, 9 aa, synthetic construct
GGKGHDLLN

SEQ ID NO: 12394 - protein, 9 aa, synthetic construct
GGVGNDVIT

SEQ ID NO: 12395 - protein, 9 aa, synthetic construct
GGGGRDTAS

SEQ ID NO: 12396 - protein, 9 aa, synthetic construct
GGIGADILR

SEQ ID NO: 12397 - protein, 9 aa, synthetic construct
GGAGTDSLY

SEQ ID NO: 12398 - protein, 9 aa, synthetic construct
GGEGDDSLV

SEQ ID NO: 12399 - protein, 9 aa, synthetic construct
GGLGDDLIS

SEQ ID NO: 12400 - protein, 9 aa, synthetic construct
GGEGSDTLN

SEQ ID NO: 12401 - protein, 9 aa, synthetic construct
GGEGGDSLA

SEQ ID NO: 12402 - protein, 9 aa, synthetic construct
GGDGDDTVS

SEQ ID NO: 12403 - protein, 9 aa, synthetic construct
GGVGNDVFY

SEQ ID NO: 12404 - protein, 9 aa, synthetic construct
GGLGDDLFI

SEQ ID NO: 12405 - protein, 9 aa, synthetic construct
GGGGNDHLD

SEQ ID NO: 12406 - protein, 9 aa, synthetic construct
GGDGDDEIF

SEQ ID NO: 12407 - protein, 9 aa, synthetic construct
GGDGSDVIN

SEQ ID NO: 12408 - protein, 9 aa, synthetic construct
GGKGADRLS

SEQ ID NO: 12409 - protein, 9 aa, synthetic construct
GGQGWDTLD

SEQ ID NO: 12410 - protein, 9 aa, synthetic construct
GGTGTDVLF

SEQ ID NO: 12411 - protein, 9 aa, synthetic construct
GGMGNDIIY

SEQ ID NO: 12412 - protein, 9 aa, synthetic construct
GGDGNDSYY

SEQ ID NO: 12413 - protein, 9 aa, synthetic construct
GGLGHDVVS

SEQ ID NO: 12414 - protein, 9 aa, synthetic construct
GGAGDDTAS

SEQ ID NO: 12415 - protein, 9 aa, synthetic construct
GGDGSDVFR

SEQ ID NO: 12416 - protein, 9 aa, synthetic construct
GGQGVDWLY

SEQ ID NO: 12417 - protein, 9 aa, synthetic construct
GGEGNDVLM

SEQ ID NO: 12418 - protein, 9 aa, synthetic construct
GGLGDDKLI

SEQ ID NO: 12419 - protein, 9 aa, synthetic construct
GGDGGDSIL

SEQ ID NO: 12420 - protein, 9 aa, synthetic construct
GGAGRDVML

SEQ ID NO: 12421 - protein, 9 aa, synthetic construct
GGGGLDRLF

SEQ ID NO: 12422 - protein, 9 aa, synthetic construct
GGPGSDTLI

SEQ ID NO: 12423 - protein, 9 aa, synthetic construct
GGAGRDVMS

SEQ ID NO: 12424 - protein, 9 aa, synthetic construct
GGQGVDTLT

SEQ ID NO: 12425 - protein, 9 aa, synthetic construct
GGNGDDTVQ

SEQ ID NO: 12426 - protein, 9 aa, synthetic construct
GGAGDDTAD

SEQ ID NO: 12427 - protein, 9 aa, synthetic construct
GGAGRDVYH

SEQ ID NO: 12428 - protein, 9 aa, synthetic construct
GGTGTDYLY

SEQ ID NO: 12429 - protein, 9 aa, synthetic construct
GGNGIDTLD

SEQ ID NO: 12430 - protein, 9 aa, synthetic construct
GGAGKDILS

SEQ ID NO: 12431 - protein, 9 aa, synthetic construct
GGLGDDLIV

SEQ ID NO: 12432 - protein, 9 aa, synthetic construct
GGLGHDTLV

SEQ ID NO: 12433 - protein, 9 aa, synthetic construct
GGDGGDSLD

SEQ ID NO: 12434 - protein, 9 aa, synthetic construct
GGDGSDVLT

SEQ ID NO: 12435 - protein, 9 aa, synthetic construct
GGLGHDSMF

SEQ ID NO: 12436 - protein, 9 aa, synthetic construct
GGTGVDTMV

SEQ ID NO: 12437 - protein, 9 aa, synthetic construct
GGLGHDSLT

SEQ ID NO: 12438 - protein, 9 aa, synthetic construct
GGDGSDVLL

SEQ ID NO: 12439 - protein, 9 aa, synthetic construct
GGTGVDTVD

SEQ ID NO: 12440 - protein, 9 aa, synthetic construct
GGDGNDTAN

SEQ ID NO: 12441 - protein, 9 aa, synthetic construct
GGEGSDTLE

SEQ ID NO: 12442 - protein, 9 aa, synthetic construct
GGQGSDTID

SEQ ID NO: 12443 - protein, 9 aa, synthetic construct
GGDGMDILS

SEQ ID NO: 12444 - protein, 9 aa, synthetic construct
GGAGDDSFD

SEQ ID NO: 12445 - protein, 9 aa, synthetic construct
GGTGVDVMT

SEQ ID NO: 12446 - protein, 9 aa, synthetic construct
GGVGNDTMV

SEQ ID NO: 12447 - protein, 9 aa, synthetic construct
GGTGVDQFR

SEQ ID NO: 12448 - protein, 9 aa, synthetic construct
GGLGDDLMY

SEQ ID NO: 12449 - protein, 9 aa, synthetic construct
GGNGDDIYL

SEQ ID NO: 12450 - protein, 9 aa, synthetic construct
GGVGNDTMT

SEQ ID NO: 12451 - protein, 9 aa, synthetic construct
GGAGTDRLI

SEQ ID NO: 12452 - protein, 9 aa, synthetic construct
GGAGDDRYT

SEQ ID NO: 12453 - protein, 9 aa, synthetic construct
GGVGNDTMR

SEQ ID NO: 12454 - protein, 9 aa, synthetic construct
GGVGNDTMI

SEQ ID NO: 12455 - protein, 9 aa, synthetic construct
GGMGSDLLL

SEQ ID NO: 12456 - protein, 9 aa, synthetic construct
GGGGRDSLS

SEQ ID NO: 12457 - protein, 9 aa, synthetic construct
GGTGVDYMA

SEQ ID NO: 12458 - protein, 9 aa, synthetic construct
GGDGSDVMS

SEQ ID NO: 12459 - protein, 9 aa, synthetic construct
GGAGDDSIA

SEQ ID NO: 12460 - protein, 9 aa, synthetic construct
GGVGNDTVY

SEQ ID NO: 12461 - protein, 9 aa, synthetic construct
GGGGRDSLW

SEQ ID NO: 12462 - protein, 9 aa, synthetic construct
GGAGTDRVS

SEQ ID NO: 12463 - protein, 9 aa, synthetic construct
GGTGVDQLT

SEQ ID NO: 12464 - protein, 9 aa, synthetic construct
GGAGTDSLL

SEQ ID NO: 12465 - protein, 9 aa, synthetic construct
GGAGSDAFI

SEQ ID NO: 12466 - protein, 9 aa, synthetic construct
GGLGHDTLR

SEQ ID NO: 12467 - protein, 9 aa, synthetic construct
GGAGTDSLD

SEQ ID NO: 12468 - protein, 9 aa, synthetic construct
GGDGDDEAF

SEQ ID NO: 12469 - protein, 9 aa, synthetic construct
GGAGTDSIT

SEQ ID NO: 12470 - protein, 9 aa, synthetic construct
GGIGADHLI

SEQ ID NO: 12471 - protein, 9 aa, synthetic construct
GGGGADRLW

SEQ ID NO: 12472 - protein, 9 aa, synthetic construct
GGAGSDALF

SEQ ID NO: 12473 - protein, 9 aa, synthetic construct
GGDGSDVLF

SEQ ID NO: 12474 - protein, 9 aa, synthetic construct
GGLGHDTLL

SEQ ID NO: 12475 - protein, 9 aa, synthetic construct
GGAGSDALL

SEQ ID NO: 12476 - protein, 9 aa, synthetic construct
GGSGNDSII

SEQ ID NO: 12477 - protein, 9 aa, synthetic construct
GGLGDDLLK

SEQ ID NO: 12478 - protein, 9 aa, synthetic construct
GGLGHDTLI

SEQ ID NO: 12479 - protein, 9 aa, synthetic construct
GGAGDDSIQ

SEQ ID NO: 12480 - protein, 9 aa, synthetic construct
GGAGSDAMA

SEQ ID NO: 12481 - protein, 9 aa, synthetic construct
GGDGQDIAH

SEQ ID NO: 12482 - protein, 9 aa, synthetic construct
GGLGHDTLA

SEQ ID NO: 12483 - protein, 9 aa, synthetic construct
GGAGKDILK

SEQ ID NO: 12484 - protein, 9 aa, synthetic construct
GGGGADRMY

SEQ ID NO: 12485 - protein, 9 aa, synthetic construct
GGLGDDLLY

SEQ ID NO: 12486 - protein, 9 aa, synthetic construct
GGEGSDTYV

SEQ ID NO: 12487 - protein, 9 aa, synthetic construct
GGLGEDRLY

SEQ ID NO: 12488 - protein, 9 aa, synthetic construct
GGSGDDDME

SEQ ID NO: 12489 - protein, 9 aa, synthetic construct
GGSGDDTVR

SEQ ID NO: 12490 - protein, 9 aa, synthetic construct
GGTGDDTVN

SEQ ID NO: 12491 - protein, 9 aa, synthetic construct
GGDGADHLI

SEQ ID NO: 12492 - protein, 9 aa, synthetic construct
GGSGDDTVI

SEQ ID NO: 12493 - protein, 9 aa, synthetic construct
GGSGHDVLN

SEQ ID NO: 12494 - protein, 9 aa, synthetic construct
GGNGDDGLD

SEQ ID NO: 12495 - protein, 9 aa, synthetic construct
GGTGADSLE

SEQ ID NO: 12496 - protein, 9 aa, synthetic construct
GGEGRDALY

SEQ ID NO: 12497 - protein, 9 aa, synthetic construct
GGTGDDTVG

SEQ ID NO: 12498 - protein, 9 aa, synthetic construct
GGTGDDTVF

SEQ ID NO: 12499 - protein, 9 aa, synthetic construct
GGDGADIFR

SEQ ID NO: 12500 - protein, 9 aa, synthetic construct
GGEGYDILN

SEQ ID NO: 12501 - protein, 9 aa, synthetic construct
GGSGGDTLL

SEQ ID NO: 12502 - protein, 9 aa, synthetic construct
GGSGHDVLT

SEQ ID NO: 12503 - protein, 9 aa, synthetic construct
GGDGADHIS

SEQ ID NO: 12504 - protein, 9 aa, synthetic construct
GGNGVDKID

SEQ ID NO: 12505 - protein, 9 aa, synthetic construct
GGGGNDYLF

SEQ ID NO: 12506 - protein, 9 aa, synthetic construct
GGNGVDKLD

SEQ ID NO: 12507 - protein, 9 aa, synthetic construct
GGSGADSLA

SEQ ID NO: 12508 - protein, 9 aa, synthetic construct
GGNGVDDLW

SEQ ID NO: 12509 - protein, 9 aa, synthetic construct
GGTGDDTYH

SEQ ID NO: 12510 - protein, 9 aa, synthetic construct
GGAGKDSLT

SEQ ID NO: 12511 - protein, 9 aa, synthetic construct
GGAGGDFLI

SEQ ID NO: 12512 - protein, 9 aa, synthetic construct
GGDGEDQLF

SEQ ID NO: 12513 - protein, 9 aa, synthetic construct
GGTGDDVIE

SEQ ID NO: 12514 - protein, 9 aa, synthetic construct
GGSGRDSIV

SEQ ID NO: 12515 - protein, 9 aa, synthetic construct
GGIGRDSLS

SEQ ID NO: 12516 - protein, 9 aa, synthetic construct
GGKGDDSLN

SEQ ID NO: 12517 - protein, 9 aa, synthetic construct
GGKGRDRME

SEQ ID NO: 12518 - protein, 9 aa, synthetic construct
GGSGGDTLN

SEQ ID NO: 12519 - protein, 9 aa, synthetic construct
GGYGDDSLD

SEQ ID NO: 12520 - protein, 9 aa, synthetic construct
GGAGADKMA

SEQ ID NO: 12521 - protein, 9 aa, synthetic construct
GGYGDDSID

SEQ ID NO: 12522 - protein, 9 aa, synthetic construct
GGIGNDTYR

SEQ ID NO: 12523 - protein, 9 aa, synthetic construct
GGEGNDHLN

SEQ ID NO: 12524 - protein, 9 aa, synthetic construct
GGTGDDVAY

SEQ ID NO: 12525 - protein, 9 aa, synthetic construct
GGDGDDLMQ

SEQ ID NO: 12526 - protein, 9 aa, synthetic construct
GGSGDDTVA

SEQ ID NO: 12527 - protein, 9 aa, synthetic construct
GGLGNDRLM

SEQ ID NO: 12528 - protein, 9 aa, synthetic construct
GGNGQDTLL

SEQ ID NO: 12529 - protein, 9 aa, synthetic construct
GGAGNDTMG

SEQ ID NO: 12530 - protein, 9 aa, synthetic construct
GGDGRDTVK

SEQ ID NO: 12531 - protein, 9 aa, synthetic construct
GGDGRDTVL

SEQ ID NO: 12532 - protein, 9 aa, synthetic construct
GGTGDDTMA

SEQ ID NO: 12533 - protein, 9 aa, synthetic construct
GGLGNDRIW

SEQ ID NO: 12534 - protein, 9 aa, synthetic construct
GGTGDDTLM

SEQ ID NO: 12535 - protein, 9 aa, synthetic construct
GGIGLDTLR

SEQ ID NO: 12536 - protein, 9 aa, synthetic construct
GGTGKDSYV

SEQ ID NO: 12537 - protein, 9 aa, synthetic construct
GGYGNDTII

SEQ ID NO: 12538 - protein, 9 aa, synthetic construct
GGGGSDTIT

SEQ ID NO: 12539 - protein, 9 aa, synthetic construct
GGKGNDIIY

SEQ ID NO: 12540 - protein, 9 aa, synthetic construct
GGSGDDVFT

SEQ ID NO: 12541 - protein, 9 aa, synthetic construct
GGLGNDRIS

SEQ ID NO: 12542 - protein, 9 aa, synthetic construct
GGTGDDDLH

SEQ ID NO: 12543 - protein, 9 aa, synthetic construct
GGGGHDTLS

SEQ ID NO: 12544 - protein, 9 aa, synthetic construct
GGDGNDRLG

SEQ ID NO: 12545 - protein, 9 aa, synthetic construct
GGAGGDCFL

SEQ ID NO: 12546 - protein, 9 aa, synthetic construct
GGNGNDRLA

SEQ ID NO: 12547 - protein, 9 aa, synthetic construct
GGAGADLFA

SEQ ID NO: 12548 - protein, 9 aa, synthetic construct
GGAGADLFD

SEQ ID NO: 12549 - protein, 9 aa, synthetic construct
GGSGQDIFH

SEQ ID NO: 12550 - protein, 9 aa, synthetic construct
GGNGVDRLN

SEQ ID NO: 12551 - protein, 9 aa, synthetic construct
GGSGRDELH

SEQ ID NO: 12552 - protein, 9 aa, synthetic construct
GGTGDDTMY

SEQ ID NO: 12553 - protein, 9 aa, synthetic construct
GGAGGDDLS

SEQ ID NO: 12554 - protein, 9 aa, synthetic construct
GGKGNDTLH

SEQ ID NO: 12555 - protein, 9 aa, synthetic construct
GGSGGDTLH

SEQ ID NO: 12556 - protein, 9 aa, synthetic construct
GGSGADSIL

SEQ ID NO: 12557 - protein, 9 aa, synthetic construct
GGSGGDTLF

SEQ ID NO: 12558 - protein, 9 aa, synthetic construct
GGDGEDTLV

SEQ ID NO: 12559 - protein, 9 aa, synthetic construct
GGSGDDTYY

SEQ ID NO: 12560 - protein, 9 aa, synthetic construct
GGSGADSIF

SEQ ID NO: 12561 - protein, 9 aa, synthetic construct
GGAGLDLLY

SEQ ID NO: 12562 - protein, 9 aa, synthetic construct
GGLGSDKLT

SEQ ID NO: 12563 - protein, 9 aa, synthetic construct
GGEGNDMLY

SEQ ID NO: 12564 - protein, 9 aa, synthetic construct
GGAGADKVN

SEQ ID NO: 12565 - protein, 9 aa, synthetic construct
GGEGYDELY

SEQ ID NO: 12566 - protein, 9 aa, synthetic construct
GGNGNDSLA

SEQ ID NO: 12567 - protein, 9 aa, synthetic construct
GGGGDDVVT

SEQ ID NO: 12568 - protein, 9 aa, synthetic construct
GGAGHDKIE

SEQ ID NO: 12569 - protein, 9 aa, synthetic construct
GGAGADKVY

SEQ ID NO: 12570 - protein, 9 aa, synthetic construct
GGSGQDILI

SEQ ID NO: 12571 - protein, 9 aa, synthetic construct
GGDGEDTLS

SEQ ID NO: 12572 - protein, 9 aa, synthetic construct
GGAGGDHLD

SEQ ID NO: 12573 - protein, 9 aa, synthetic construct
GGAGFDTIE

SEQ ID NO: 12574 - protein, 9 aa, synthetic construct
GGEGNDLVG

SEQ ID NO: 12575 - protein, 9 aa, synthetic construct
GGSGADTVI

SEQ ID NO: 12576 - protein, 9 aa, synthetic construct
GGTGIDSIA

SEQ ID NO: 12577 - protein, 9 aa, synthetic construct
GGYGNDRLY

SEQ ID NO: 12578 - protein, 9 aa, synthetic construct
GGKGRDRLA

SEQ ID NO: 12579 - protein, 9 aa, synthetic construct
GGNGTDRAS

SEQ ID NO: 12580 - protein, 9 aa, synthetic construct
GGDGRDTIN

SEQ ID NO: 12581 - protein, 9 aa, synthetic construct
GGTGDDWLA

SEQ ID NO: 12582 - protein, 9 aa, synthetic construct
GGTGADTFF

SEQ ID NO: 12583 - protein, 9 aa, synthetic construct
GGIGSDKLT

SEQ ID NO: 12584 - protein, 9 aa, synthetic construct
GGTGDDVIH

SEQ ID NO: 12585 - protein, 9 aa, synthetic construct
GGLGNDVFA

SEQ ID NO: 12586 - protein, 9 aa, synthetic construct
GGYGDDTLL

SEQ ID NO: 12587 - protein, 9 aa, synthetic construct
GGDGNDWLH

SEQ ID NO: 12588 - protein, 9 aa, synthetic construct
GGSGADTMM

SEQ ID NO: 12589 - protein, 9 aa, synthetic construct
GGSGDDTIF

SEQ ID NO: 12590 - protein, 9 aa, synthetic construct
GGGGEDLLN

SEQ ID NO: 12591 - protein, 9 aa, synthetic construct
GGDGFDTAS

SEQ ID NO: 12592 - protein, 9 aa, synthetic construct
GGLGSDTYR

SEQ ID NO: 12593 - protein, 9 aa, synthetic construct
GGDGADILA

SEQ ID NO: 12594 - protein, 9 aa, synthetic construct
GGYGNDRLV

SEQ ID NO: 12595 - protein, 9 aa, synthetic construct
GGGGSDTLM

SEQ ID NO: 12596 - protein, 9 aa, synthetic construct
GGDGADILE

SEQ ID NO: 12597 - protein, 9 aa, synthetic construct
GGYGDDTYI

SEQ ID NO: 12598 - protein, 9 aa, synthetic construct
GGKGDDHLE

SEQ ID NO: 12599 - protein, 9 aa, synthetic construct
GGAGNDQMT

SEQ ID NO: 12600 - protein, 9 aa, synthetic construct
GGSGGDVIT

SEQ ID NO: 12601 - protein, 9 aa, synthetic construct
GGYGDDTVF

SEQ ID NO: 12602 - protein, 9 aa, synthetic construct
GGDGADRLQ

SEQ ID NO: 12603 - protein, 9 aa, synthetic construct
GGSGADVFE

SEQ ID NO: 12604 - protein, 9 aa, synthetic construct
GGTGDDYIE

SEQ ID NO: 12605 - protein, 9 aa, synthetic construct
GGAGADFLD

SEQ ID NO: 12606 - protein, 9 aa, synthetic construct
GGTGIDQMS

SEQ ID NO: 12607 - protein, 9 aa, synthetic construct
GGAGNDQMN

SEQ ID NO: 12608 - protein, 9 aa, synthetic construct
GGFGADTMI

SEQ ID NO: 12609 - protein, 9 aa, synthetic construct
GGYGDDTLV

SEQ ID NO: 12610 - protein, 9 aa, synthetic construct
GGLGNDRYV

SEQ ID NO: 12611 - protein, 9 aa, synthetic construct
GGDGHDLLI

SEQ ID NO: 12612 - protein, 9 aa, synthetic construct
GGSGSDAFV

SEQ ID NO: 12613 - protein, 9 aa, synthetic construct
GGEGYDVFK

SEQ ID NO: 12614 - protein, 9 aa, synthetic construct
GGIGNDTVA

SEQ ID NO: 12615 - protein, 9 aa, synthetic construct
GGFGDDLIS

SEQ ID NO: 12616 - protein, 9 aa, synthetic construct
GGDGDDRFI

SEQ ID NO: 12617 - protein, 9 aa, synthetic construct
GGTGIDTMV

SEQ ID NO: 12618 - protein, 9 aa, synthetic construct
GGYGNDSIS

SEQ ID NO: 12619 - protein, 9 aa, synthetic construct
GGNGTDTLD

SEQ ID NO: 12620 - protein, 9 aa, synthetic construct
GGIGNDELF

SEQ ID NO: 12621 - protein, 9 aa, synthetic construct
GGSGADTIL

SEQ ID NO: 12622 - protein, 9 aa, synthetic construct
GGSGADTII

SEQ ID NO: 12623 - protein, 9 aa, synthetic construct
GGIGNDTVY

SEQ ID NO: 12624 - protein, 9 aa, synthetic construct
GGSGADTIF

SEQ ID NO: 12625 - protein, 9 aa, synthetic construct
GGNGTDTLL

SEQ ID NO: 12626 - protein, 9 aa, synthetic construct
GGAGNDKIG

SEQ ID NO: 12627 - protein, 9 aa, synthetic construct
GGTGIDVLT

SEQ ID NO: 12628 - protein, 9 aa, synthetic construct
GGYGNDSLF

SEQ ID NO: 12629 - protein, 9 aa, synthetic construct
GGTGDDVLA

SEQ ID NO: 12630 - protein, 9 aa, synthetic construct
GGIGNDEAQ

SEQ ID NO: 12631 - protein, 9 aa, synthetic construct
GGYGNDSLS

SEQ ID NO: 12632 - protein, 9 aa, synthetic construct
GGNGTDTLT

SEQ ID NO: 12633 - protein, 9 aa, synthetic construct
GGEGADIFA

SEQ ID NO: 12634 - protein, 9 aa, synthetic construct
GGEGDDYLN

SEQ ID NO: 12635 - protein, 9 aa, synthetic construct
GGNGTDTIN

SEQ ID NO: 12636 - protein, 9 aa, synthetic construct
GGSGADTIY

SEQ ID NO: 12637 - protein, 9 aa, synthetic construct
GGAGHDILG

SEQ ID NO: 12638 - protein, 9 aa, synthetic construct
GGIGNDEVQ

SEQ ID NO: 12639 - protein, 9 aa, synthetic construct
GGGGNDYIE

SEQ ID NO: 12640 - protein, 9 aa, synthetic construct
GGSGDDTIQ

SEQ ID NO: 12641 - protein, 9 aa, synthetic construct
GGTGDDVVS

SEQ ID NO: 12642 - protein, 9 aa, synthetic construct
GGNGRDDLR

SEQ ID NO: 12643 - protein, 9 aa, synthetic construct
GGKGDDSLD

SEQ ID NO: 12644 - protein, 9 aa, synthetic construct
GGYGDDTLA

SEQ ID NO: 12645 - protein, 9 aa, synthetic construct
GGAGGDILQ

SEQ ID NO: 12646 - protein, 9 aa, synthetic construct
GGSGQDLLT

SEQ ID NO: 12647 - protein, 9 aa, synthetic construct
GGNGTDTAD

SEQ ID NO: 12648 - protein, 9 aa, synthetic construct
GGGGEDNLN

SEQ ID NO: 12649 - protein, 9 aa, synthetic construct
GGNGNDSIV

SEQ ID NO: 12650 - protein, 9 aa, synthetic construct
GGTGIDTLN

SEQ ID NO: 12651 - protein, 9 aa, synthetic construct
GGAGNDKID

SEQ ID NO: 12652 - protein, 9 aa, synthetic construct
GGAGNDKIE

SEQ ID NO: 12653 - protein, 9 aa, synthetic construct
GGTGIDTLS

SEQ ID NO: 12654 - protein, 9 aa, synthetic construct
GGDGNDRIV

SEQ ID NO: 12655 - protein, 9 aa, synthetic construct
GGTGIDTMI

SEQ ID NO: 12656 - protein, 9 aa, synthetic construct
GGSGADRLN

SEQ ID NO: 12657 - protein, 9 aa, synthetic construct
GGSGDDVFY

SEQ ID NO: 12658 - protein, 9 aa, synthetic construct
GGSGADRLM

SEQ ID NO: 12659 - protein, 9 aa, synthetic construct
GGNGYDTIR

SEQ ID NO: 12660 - protein, 9 aa, synthetic construct
GGKGDDTID

SEQ ID NO: 12661 - protein, 9 aa, synthetic construct
GGAGNDHIE

SEQ ID NO: 12662 - protein, 9 aa, synthetic construct
GGEGADTID

SEQ ID NO: 12663 - protein, 9 aa, synthetic construct
GGAGFDVAV

SEQ ID NO: 12664 - protein, 9 aa, synthetic construct
GGKGDDLLL

SEQ ID NO: 12665 - protein, 9 aa, synthetic construct
GGTGDDELH

SEQ ID NO: 12666 - protein, 9 aa, synthetic construct
GGKGDDTIF

SEQ ID NO: 12667 - protein, 9 aa, synthetic construct
GGDGFDTIY

SEQ ID NO: 12668 - protein, 9 aa, synthetic construct
GGEGNDHLD

SEQ ID NO: 12669 - protein, 9 aa, synthetic construct
GGSGADRLL

SEQ ID NO: 12670 - protein, 9 aa, synthetic construct
GGSGADLLN

SEQ ID NO: 12671 - protein, 9 aa, synthetic construct
GGAGHDLLK

SEQ ID NO: 12672 - protein, 9 aa, synthetic construct
GGEGIDTAS

SEQ ID NO: 12673 - protein, 9 aa, synthetic construct
GGTGDDRMT

SEQ ID NO: 12674 - protein, 9 aa, synthetic construct
GGIGIDSLF

SEQ ID NO: 12675 - protein, 9 aa, synthetic construct
GGDGQDTII

SEQ ID NO: 12676 - protein, 9 aa, synthetic construct
GGTGDDELL

SEQ ID NO: 12677 - protein, 9 aa, synthetic construct
GGEGIDTFI

SEQ ID NO: 12678 - protein, 9 aa, synthetic construct
GGNGYDQLD

SEQ ID NO: 12679 - protein, 9 aa, synthetic construct
GGDGADVFL

SEQ ID NO: 12680 - protein, 9 aa, synthetic construct
GGDGGDLLL

SEQ ID NO: 12681 - protein, 9 aa, synthetic construct
GGSGDDWLE

SEQ ID NO: 12682 - protein, 9 aa, synthetic construct
GGYGNDVLT

SEQ ID NO: 12683 - protein, 9 aa, synthetic construct
GGYGDDHLK

SEQ ID NO: 12684 - protein, 9 aa, synthetic construct
GGKGNDTII

SEQ ID NO: 12685 - protein, 9 aa, synthetic construct
GGAGLDNLD

SEQ ID NO: 12686 - protein, 9 aa, synthetic construct
GGYGNDVLV

SEQ ID NO: 12687 - protein, 9 aa, synthetic construct
GGSGQDEIN

SEQ ID NO: 12688 - protein, 9 aa, synthetic construct
GGNGYDIAD

SEQ ID NO: 12689 - protein, 9 aa, synthetic construct
GGNGYDILI

SEQ ID NO: 12690 - protein, 9 aa, synthetic construct
GGAGADLLK

SEQ ID NO: 12691 - protein, 9 aa, synthetic construct
GGDGDDIYV

SEQ ID NO: 12692 - protein, 9 aa, synthetic construct
GGMGDDRLD

SEQ ID NO: 12693 - protein, 9 aa, synthetic construct
GGAGNDVFI

SEQ ID NO: 12694 - protein, 9 aa, synthetic construct
GGYGNDVLW

SEQ ID NO: 12695 - protein, 9 aa, synthetic construct
GGAGFDVLK

SEQ ID NO: 12696 - protein, 9 aa, synthetic construct
GGKGDDELY

SEQ ID NO: 12697 - protein, 9 aa, synthetic construct
GGGGDDVIV

SEQ ID NO: 12698 - protein, 9 aa, synthetic construct
GGAGKDYLN

SEQ ID NO: 12699 - protein, 9 aa, synthetic construct
GGNGYDVLI

SEQ ID NO: 12700 - protein, 9 aa, synthetic construct
GGGGDDVII

SEQ ID NO: 12701 - protein, 9 aa, synthetic construct
GGNGNDYLY

SEQ ID NO: 12702 - protein, 9 aa, synthetic construct
GGYGADVLD

SEQ ID NO: 12703 - protein, 9 aa, synthetic construct
GGTGDDELY

SEQ ID NO: 12704 - protein, 9 aa, synthetic construct
GGDGADDLF

SEQ ID NO: 12705 - protein, 9 aa, synthetic construct
GGTGDDRLK

SEQ ID NO: 12706 - protein, 9 aa, synthetic construct
GGSGRDRLV

SEQ ID NO: 12707 - protein, 9 aa, synthetic construct
GGEGDDLIG

SEQ ID NO: 12708 - protein, 9 aa, synthetic construct
GGAGADLMV

SEQ ID NO: 12709 - protein, 9 aa, synthetic construct
GGAGFDTIS

SEQ ID NO: 12710 - protein, 9 aa, synthetic construct
GGEGNDQIF

SEQ ID NO: 12711 - protein, 9 aa, synthetic construct
GGKGNDSLN

SEQ ID NO: 12712 - protein, 9 aa, synthetic construct
GGDGDDKIA

SEQ ID NO: 12713 - protein, 9 aa, synthetic construct
GGNGNDQMI

SEQ ID NO: 12714 - protein, 9 aa, synthetic construct
GGSGGDRLE

SEQ ID NO: 12715 - protein, 9 aa, synthetic construct
GGSGRDRLT

SEQ ID NO: 12716 - protein, 9 aa, synthetic construct
GGNGNDYIS

SEQ ID NO: 12717 - protein, 9 aa, synthetic construct
GGPGADIFQ

SEQ ID NO: 12718 - protein, 9 aa, synthetic construct
GGGGTDTIS

SEQ ID NO: 12719 - protein, 9 aa, synthetic construct
GGLGYDQLS

SEQ ID NO: 12720 - protein, 9 aa, synthetic construct
GGKGDDLLH

SEQ ID NO: 12721 - protein, 9 aa, synthetic construct
GGDGHDIIS

SEQ ID NO: 12722 - protein, 9 aa, synthetic construct
GGTGDDRMR

SEQ ID NO: 12723 - protein, 9 aa, synthetic construct
GGDGADTAI

SEQ ID NO: 12724 - protein, 9 aa, synthetic construct
GGAGNDVFS

SEQ ID NO: 12725 - protein, 9 aa, synthetic construct
GGAGFDTVI

SEQ ID NO: 12726 - protein, 9 aa, synthetic construct
GGAGFDTVD

SEQ ID NO: 12727 - protein, 9 aa, synthetic construct
GGAGADLMR

SEQ ID NO: 12728 - protein, 9 aa, synthetic construct
GGTGADRFS

SEQ ID NO: 12729 - protein, 9 aa, synthetic construct
GGTGLDTLV

SEQ ID NO: 12730 - protein, 9 aa, synthetic construct
GGAGFDTMS

SEQ ID NO: 12731 - protein, 9 aa, synthetic construct
GGYGNDVYV

SEQ ID NO: 12732 - protein, 9 aa, synthetic construct
GGSGGDRLS

SEQ ID NO: 12733 - protein, 9 aa, synthetic construct
GGFGDDLYI

SEQ ID NO: 12734 - protein, 9 aa, synthetic construct
GGAGADELV

SEQ ID NO: 12735 - protein, 9 aa, synthetic construct
GGTGLDVID

SEQ ID NO: 12736 - protein, 9 aa, synthetic construct
GGGGTDTFV

SEQ ID NO: 12737 - protein, 9 aa, synthetic construct
GGTGDDRME

SEQ ID NO: 12738 - protein, 9 aa, synthetic construct
GGAGHDLLM

SEQ ID NO: 12739 - protein, 9 aa, synthetic construct
GGTGDDRLW

SEQ ID NO: 12740 - protein, 9 aa, synthetic construct
GGDGADTAD

SEQ ID NO: 12741 - protein, 9 aa, synthetic construct
GGSGGDSLF

SEQ ID NO: 12742 - protein, 9 aa, synthetic construct
GGEGNDNLS

SEQ ID NO: 12743 - protein, 9 aa, synthetic construct
GGAGNDVAS

SEQ ID NO: 12744 - protein, 9 aa, synthetic construct
GGEGMDLFT

SEQ ID NO: 12745 - protein, 9 aa, synthetic construct
GGDGNDVIM

SEQ ID NO: 12746 - protein, 9 aa, synthetic construct
GGAGKDVFA

SEQ ID NO: 12747 - protein, 9 aa, synthetic construct
GGTGDDSYF

SEQ ID NO: 12748 - protein, 9 aa, synthetic construct
GGAGADEVL

SEQ ID NO: 12749 - protein, 9 aa, synthetic construct
GGDGADSLG

SEQ ID NO: 12750 - protein, 9 aa, synthetic construct
GGDGRDVLS

SEQ ID NO: 12751 - protein, 9 aa, synthetic construct
GGDGNDVVD

SEQ ID NO: 12752 - protein, 9 aa, synthetic construct
GGAGGDALF

SEQ ID NO: 12753 - protein, 9 aa, synthetic construct
GGEGQDYLL

SEQ ID NO: 12754 - protein, 9 aa, synthetic construct
GGNGADTII

SEQ ID NO: 12755 - protein, 9 aa, synthetic construct
GGSGADRFF

SEQ ID NO: 12756 - protein, 9 aa, synthetic construct
GGDGFDSLL

SEQ ID NO: 12757 - protein, 9 aa, synthetic construct
GGMGADVLD

SEQ ID NO: 12758 - protein, 9 aa, synthetic construct
GGAGIDALN

SEQ ID NO: 12759 - protein, 9 aa, synthetic construct
GGAGNDKIV

SEQ ID NO: 12760 - protein, 9 aa, synthetic construct
GGTGDDSMD

SEQ ID NO: 12761 - protein, 9 aa, synthetic construct
GGTGDDSMA

SEQ ID NO: 12762 - protein, 9 aa, synthetic construct
GGAGNDHLL

SEQ ID NO: 12763 - protein, 9 aa, synthetic construct
GGSGDDVIW

SEQ ID NO: 12764 - protein, 9 aa, synthetic construct
GGFGHDSLN

SEQ ID NO: 12765 - protein, 9 aa, synthetic construct
GGSGDDVIT

SEQ ID NO: 12766 - protein, 9 aa, synthetic construct
GGSGDDVIA

SEQ ID NO: 12767 - protein, 9 aa, synthetic construct
GGDGADSIQ

SEQ ID NO: 12768 - protein, 9 aa, synthetic construct
GGYGDDNLF

SEQ ID NO: 12769 - protein, 9 aa, synthetic construct
GGDGADSIR

SEQ ID NO: 12770 - protein, 9 aa, synthetic construct
GGAGNDTVH

SEQ ID NO: 12771 - protein, 9 aa, synthetic construct
GGEGNDNIL

SEQ ID NO: 12772 - protein, 9 aa, synthetic construct
GGTGKDTLS

SEQ ID NO: 12773 - protein, 9 aa, synthetic construct
GGFGDDLLS

SEQ ID NO: 12774 - protein, 9 aa, synthetic construct
GGTGDDTFY

SEQ ID NO: 12775 - protein, 9 aa, synthetic construct
GGNGNDRIS

SEQ ID NO: 12776 - protein, 9 aa, synthetic construct
GGDGADSIT

SEQ ID NO: 12777 - protein, 9 aa, synthetic construct
GGAGADLIA

SEQ ID NO: 12778 - protein, 9 aa, synthetic construct
GGGGSDKMS

SEQ ID NO: 12779 - protein, 9 aa, synthetic construct
GGAGNDQIW

SEQ ID NO: 12780 - protein, 9 aa, synthetic construct
GGAGKDTYV

SEQ ID NO: 12781 - protein, 9 aa, synthetic construct
GGAGGDALY

SEQ ID NO: 12782 - protein, 9 aa, synthetic construct
GGKGRDTID

SEQ ID NO: 12783 - protein, 9 aa, synthetic construct
GGGGDDVLQ

SEQ ID NO: 12784 - protein, 9 aa, synthetic construct
GGFGNDFLD

SEQ ID NO: 12785 - protein, 9 aa, synthetic construct
GGDGADELQ

SEQ ID NO: 12786 - protein, 9 aa, synthetic construct
GGGGNDLVY

SEQ ID NO: 12787 - protein, 9 aa, synthetic construct
GGEGADTII

SEQ ID NO: 12788 - protein, 9 aa, synthetic construct
GGAGNDTYS

SEQ ID NO: 12789 - protein, 9 aa, synthetic construct
GGAGADLIS

SEQ ID NO: 12790 - protein, 9 aa, synthetic construct
GGKGRDVFV

SEQ ID NO: 12791 - protein, 9 aa, synthetic construct
GGTGDDSIT

SEQ ID NO: 12792 - protein, 9 aa, synthetic construct
GGKGRDVID

SEQ ID NO: 12793 - protein, 9 aa, synthetic construct
GGSGADNLD

SEQ ID NO: 12794 - protein, 9 aa, synthetic construct
GGYGDDILN

SEQ ID NO: 12795 - protein, 9 aa, synthetic construct
GGDGRDWVR

SEQ ID NO: 12796 - protein, 9 aa, synthetic construct
GGTGDDSIS

SEQ ID NO: 12797 - protein, 9 aa, synthetic construct
GGNGWDVLG

SEQ ID NO: 12798 - protein, 9 aa, synthetic construct
GGTGDDSIN

SEQ ID NO: 12799 - protein, 9 aa, synthetic construct
GGSGDDVYN

SEQ ID NO: 12800 - protein, 9 aa, synthetic construct
GGKGRDVLN

SEQ ID NO: 12801 - protein, 9 aa, synthetic construct
GGTGDDELD

SEQ ID NO: 12802 - protein, 9 aa, synthetic construct
GGSGDDVYV

SEQ ID NO: 12803 - protein, 9 aa, synthetic construct
GGEGNDHLE

SEQ ID NO: 12804 - protein, 9 aa, synthetic construct
GGGGKDKIN

SEQ ID NO: 12805 - protein, 9 aa, synthetic construct
GGDGDDSAW

SEQ ID NO: 12806 - protein, 9 aa, synthetic construct
GGYGNDTYL

SEQ ID NO: 12807 - protein, 9 aa, synthetic construct
GGKGNDTIW

SEQ ID NO: 12808 - protein, 9 aa, synthetic construct
GGEGDDKLA

SEQ ID NO: 12809 - protein, 9 aa, synthetic construct
GGIGKDTLT

SEQ ID NO: 12810 - protein, 9 aa, synthetic construct
GGTGADRMA

SEQ ID NO: 12811 - protein, 9 aa, synthetic construct
GGTGDDSLV

SEQ ID NO: 12812 - protein, 9 aa, synthetic construct
GGGGNDYLV

SEQ ID NO: 12813 - protein, 9 aa, synthetic construct
GGEGADILY

SEQ ID NO: 12814 - protein, 9 aa, synthetic construct
GGTGDDSLM

SEQ ID NO: 12815 - protein, 9 aa, synthetic construct
GGSGGDSLT

SEQ ID NO: 12816 - protein, 9 aa, synthetic construct
GGAGADLIL

SEQ ID NO: 12817 - protein, 9 aa, synthetic construct
GGSGADQIY

SEQ ID NO: 12818 - protein, 9 aa, synthetic construct
GGAGADEMS

SEQ ID NO: 12819 - protein, 9 aa, synthetic construct
GGSGGDSLN

SEQ ID NO: 12820 - protein, 9 aa, synthetic construct
GGGGSDTFR

SEQ ID NO: 12821 - protein, 9 aa, synthetic construct
GGNGDDEMQ

SEQ ID NO: 12822 - protein, 9 aa, synthetic construct
GGNGNDRIG

SEQ ID NO: 12823 - protein, 9 aa, synthetic construct
GGGGDDVLK

SEQ ID NO: 12824 - protein, 9 aa, synthetic construct
GGSGDDVVH

SEQ ID NO: 12825 - protein, 9 aa, synthetic construct
GGTGIDNLN

SEQ ID NO: 12826 - protein, 9 aa, synthetic construct
GGTGIDMLY

SEQ ID NO: 12827 - protein, 9 aa, synthetic construct
GGGGIDAIY

SEQ ID NO: 12828 - protein, 9 aa, synthetic construct
GGLGNDTMA

SEQ ID NO: 12829 - protein, 9 aa, synthetic construct
GGDGADQLH

SEQ ID NO: 12830 - protein, 9 aa, synthetic construct
GGFGSDTLR

SEQ ID NO: 12831 - protein, 9 aa, synthetic construct
GGSGDDHLL

SEQ ID NO: 12832 - protein, 9 aa, synthetic construct
GGSGDDHLF

SEQ ID NO: 12833 - protein, 9 aa, synthetic construct
GGSGQDVFV

SEQ ID NO: 12834 - protein, 9 aa, synthetic construct
GGSGRDTLR

SEQ ID NO: 12835 - protein, 9 aa, synthetic construct
GGSGRDTLQ

SEQ ID NO: 12836 - protein, 9 aa, synthetic construct
GGAGADILF

SEQ ID NO: 12837 - protein, 9 aa, synthetic construct
GGDGNDMLG

SEQ ID NO: 12838 - protein, 9 aa, synthetic construct
GGSGDDELV

SEQ ID NO: 12839 - protein, 9 aa, synthetic construct
GGAGNDSFY

SEQ ID NO: 12840 - protein, 9 aa, synthetic construct
GGDGADLLQ

SEQ ID NO: 12841 - protein, 9 aa, synthetic construct
GGYGNDILH

SEQ ID NO: 12842 - protein, 9 aa, synthetic construct
GGNGADVLK

SEQ ID NO: 12843 - protein, 9 aa, synthetic construct
GGAGNDIVS

SEQ ID NO: 12844 - protein, 9 aa, synthetic construct
GGEGDDYIS

SEQ ID NO: 12845 - protein, 9 aa, synthetic construct
GGDGNDMLF

SEQ ID NO: 12846 - protein, 9 aa, synthetic construct
GGEGADTLG

SEQ ID NO: 12847 - protein, 9 aa, synthetic construct
GGDGRDNLA

SEQ ID NO: 12848 - protein, 9 aa, synthetic construct
GGDGQDVLL

SEQ ID NO: 12849 - protein, 9 aa, synthetic construct
GGSGHDLYV

SEQ ID NO: 12850 - protein, 9 aa, synthetic construct
GGNGNDRMY

SEQ ID NO: 12851 - protein, 9 aa, synthetic construct
GGIGNDMLT

SEQ ID NO: 12852 - protein, 9 aa, synthetic construct
GGLGSDVLI

SEQ ID NO: 12853 - protein, 9 aa, synthetic construct
GGAGADHIN

SEQ ID NO: 12854 - protein, 9 aa, synthetic construct
GGNGRDVLE

SEQ ID NO: 12855 - protein, 9 aa, synthetic construct
GGTGGDSMF

SEQ ID NO: 12856 - protein, 9 aa, synthetic construct
GGAGGDTID

SEQ ID NO: 12857 - protein, 9 aa, synthetic construct
GGGGDDYLI

SEQ ID NO: 12858 - protein, 9 aa, synthetic construct
GGKGDDRLF

SEQ ID NO: 12859 - protein, 9 aa, synthetic construct
GGAGNDIVD

SEQ ID NO: 12860 - protein, 9 aa, synthetic construct
GGIGRDYLS

SEQ ID NO: 12861 - protein, 9 aa, synthetic construct
GGIGRDVFV

SEQ ID NO: 12862 - protein, 9 aa, synthetic construct
GGSGDDIFV

SEQ ID NO: 12863 - protein, 9 aa, synthetic construct
GGAGNDIVI

SEQ ID NO: 12864 - protein, 9 aa, synthetic construct
GGSGDDIFL

SEQ ID NO: 12865 - protein, 9 aa, synthetic construct
GGEGLDTAT

SEQ ID NO: 12866 - protein, 9 aa, synthetic construct
GGSGDDIFI

SEQ ID NO: 12867 - protein, 9 aa, synthetic construct
GGYGNDHIS

SEQ ID NO: 12868 - protein, 9 aa, synthetic construct
GGAGNDSIQ

SEQ ID NO: 12869 - protein, 9 aa, synthetic construct
GGFGADILD

SEQ ID NO: 12870 - protein, 9 aa, synthetic construct
GGSGQDVLR

SEQ ID NO: 12871 - protein, 9 aa, synthetic construct
GGDGNDWIF

SEQ ID NO: 12872 - protein, 9 aa, synthetic construct
GGEGDDTLW

SEQ ID NO: 12873 - protein, 9 aa, synthetic construct
GGTGHDALT

SEQ ID NO: 12874 - protein, 9 aa, synthetic construct
GGGGNDMLF

SEQ ID NO: 12875 - protein, 9 aa, synthetic construct
GGNGSDSLD

SEQ ID NO: 12876 - protein, 9 aa, synthetic construct
GGSGQDSLT

SEQ ID NO: 12877 - protein, 9 aa, synthetic construct
GGSGHDQLY

SEQ ID NO: 12878 - protein, 9 aa, synthetic construct
GGSGRDTII

SEQ ID NO: 12879 - protein, 9 aa, synthetic construct
GGAGNDRIG

SEQ ID NO: 12880 - protein, 9 aa, synthetic construct
GGAGGDYLS

SEQ ID NO: 12881 - protein, 9 aa, synthetic construct
GGEGQDDLF

SEQ ID NO: 12882 - protein, 9 aa, synthetic construct
GGNGSDSLT

SEQ ID NO: 12883 - protein, 9 aa, synthetic construct
GGGGNDTMI

SEQ ID NO: 12884 - protein, 9 aa, synthetic construct
GGSGDDEVF

SEQ ID NO: 12885 - protein, 9 aa, synthetic construct
GGTGEDTLL

SEQ ID NO: 12886 - protein, 9 aa, synthetic construct
GGNGADVFT

SEQ ID NO: 12887 - protein, 9 aa, synthetic construct
GGAGGDRLI

SEQ ID NO: 12888 - protein, 9 aa, synthetic construct
GGAGGDRLF

SEQ ID NO: 12889 - protein, 9 aa, synthetic construct
GGDGQDVIL

SEQ ID NO: 12890 - protein, 9 aa, synthetic construct
GGSGDDQLW

SEQ ID NO: 12891 - protein, 9 aa, synthetic construct
GGLGSDVLL

SEQ ID NO: 12892 - protein, 9 aa, synthetic construct
GGSGRDTIQ

SEQ ID NO: 12893 - protein, 9 aa, synthetic construct
GGSGDDQLE

SEQ ID NO: 12894 - protein, 9 aa, synthetic construct
GGSGQDVLT

SEQ ID NO: 12895 - protein, 9 aa, synthetic construct
GGKGNDVLQ

SEQ ID NO: 12896 - protein, 9 aa, synthetic construct
GGIGNDLVF

SEQ ID NO: 12897 - protein, 9 aa, synthetic construct
GGAGNDSIW

SEQ ID NO: 12898 - protein, 9 aa, synthetic construct
GGNGADVLA

SEQ ID NO: 12899 - protein, 9 aa, synthetic construct
GGNGRDTIL

SEQ ID NO: 12900 - protein, 9 aa, synthetic construct
GGGGNDWLD

SEQ ID NO: 12901 - protein, 9 aa, synthetic construct
GGAGGDSLA

SEQ ID NO: 12902 - protein, 9 aa, synthetic construct
GGKGNDGLA

SEQ ID NO: 12903 - protein, 9 aa, synthetic construct
GGSGQDWLY

SEQ ID NO: 12904 - protein, 9 aa, synthetic construct
GGEGLDRLT

SEQ ID NO: 12905 - protein, 9 aa, synthetic construct
GGDGADLLE

SEQ ID NO: 12906 - protein, 9 aa, synthetic construct
GGEGADALD

SEQ ID NO: 12907 - protein, 9 aa, synthetic construct
GGSGDDFLH

SEQ ID NO: 12908 - protein, 9 aa, synthetic construct
GGSGDDFLG

SEQ ID NO: 12909 - protein, 9 aa, synthetic construct
GGDGADTVY

SEQ ID NO: 12910 - protein, 9 aa, synthetic construct
GGEGDDYIH

SEQ ID NO: 12911 - protein, 9 aa, synthetic construct
GGTGFDRLY

SEQ ID NO: 12912 - protein, 9 aa, synthetic construct
GGNGSDLLD

SEQ ID NO: 12913 - protein, 9 aa, synthetic construct
GGSGDDLVD

SEQ ID NO: 12914 - protein, 9 aa, synthetic construct
GGKGNDVYV

SEQ ID NO: 12915 - protein, 9 aa, synthetic construct
GGAGNDRVE

SEQ ID NO: 12916 - protein, 9 aa, synthetic construct
GGAGHDVID

SEQ ID NO: 12917 - protein, 9 aa, synthetic construct
GGAGNDRVF

SEQ ID NO: 12918 - protein, 9 aa, synthetic construct
GGEGDDRLA

SEQ ID NO: 12919 - protein, 9 aa, synthetic construct
GGAGNDIMF

SEQ ID NO: 12920 - protein, 9 aa, synthetic construct
GGAGADIFC

SEQ ID NO: 12921 - protein, 9 aa, synthetic construct
GGGGNDMLR

SEQ ID NO: 12922 - protein, 9 aa, synthetic construct
GGSGRDVFR

SEQ ID NO: 12923 - protein, 9 aa, synthetic construct
GGDGRDRID

SEQ ID NO: 12924 - protein, 9 aa, synthetic construct
GGNGSDFLM

SEQ ID NO: 12925 - protein, 9 aa, synthetic construct
GGEGIDQLF

SEQ ID NO: 12926 - protein, 9 aa, synthetic construct
GGKGNDVYI

SEQ ID NO: 12927 - protein, 9 aa, synthetic construct
GGDGADMLR

SEQ ID NO: 12928 - protein, 9 aa, synthetic construct
GGAGGDVLI

SEQ ID NO: 12929 - protein, 9 aa, synthetic construct
GGAGKDTLG

SEQ ID NO: 12930 - protein, 9 aa, synthetic construct
GGSGDDKLW

SEQ ID NO: 12931 - protein, 9 aa, synthetic construct
GGSGRDVFD

SEQ ID NO: 12932 - protein, 9 aa, synthetic construct
GGSGDDLIF

SEQ ID NO: 12933 - protein, 9 aa, synthetic construct
GGDGADQIF

SEQ ID NO: 12934 - protein, 9 aa, synthetic construct
GGEGDDYIA

SEQ ID NO: 12935 - protein, 9 aa, synthetic construct
GGDGADNLD

SEQ ID NO: 12936 - protein, 9 aa, synthetic construct
GGEGADIIL

SEQ ID NO: 12937 - protein, 9 aa, synthetic construct
GGDGEDTIN

SEQ ID NO: 12938 - protein, 9 aa, synthetic construct
GGYGKDVLT

SEQ ID NO: 12939 - protein, 9 aa, synthetic construct
GGKGNDWLD

SEQ ID NO: 12940 - protein, 9 aa, synthetic construct
GGKGNDFLN

SEQ ID NO: 12941 - protein, 9 aa, synthetic construct
GGTGFDYLN

SEQ ID NO: 12942 - protein, 9 aa, synthetic construct
GGYGKDVID

SEQ ID NO: 12943 - protein, 9 aa, synthetic construct
GGTGGDFLD

SEQ ID NO: 12944 - protein, 9 aa, synthetic construct
GGSGHDILA

SEQ ID NO: 12945 - protein, 9 aa, synthetic construct
GGGGSDILR

SEQ ID NO: 12946 - protein, 9 aa, synthetic construct
GGEGADWLY

SEQ ID NO: 12947 - protein, 9 aa, synthetic construct
GGSGDDLIT

SEQ ID NO: 12948 - protein, 9 aa, synthetic construct
GGSGRDTVL

SEQ ID NO: 12949 - protein, 9 aa, synthetic construct
GGEGADWVL

SEQ ID NO: 12950 - protein, 9 aa, synthetic construct
GGSGDDLIL

SEQ ID NO: 12951 - protein, 9 aa, synthetic construct
GGIGNDRLV

SEQ ID NO: 12952 - protein, 9 aa, synthetic construct
GGSGDDKLS

SEQ ID NO: 12953 - protein, 9 aa, synthetic construct
GGSGQDTLN

SEQ ID NO: 12954 - protein, 9 aa, synthetic construct
GGTGGDRLV

SEQ ID NO: 12955 - protein, 9 aa, synthetic construct
GGSGDDMLF

SEQ ID NO: 12956 - protein, 9 aa, synthetic construct
GGTGADVMS

SEQ ID NO: 12957 - protein, 9 aa, synthetic construct
GGAGKDTIS

SEQ ID NO: 12958 - protein, 9 aa, synthetic construct
GGSGDDMLI

SEQ ID NO: 12959 - protein, 9 aa, synthetic construct
GGSGDDMLK

SEQ ID NO: 12960 - protein, 9 aa, synthetic construct
GGSGDDMLL

SEQ ID NO: 12961 - protein, 9 aa, synthetic construct
GGKGNDYLY

SEQ ID NO: 12962 - protein, 9 aa, synthetic construct
GGAGADHLE

SEQ ID NO: 12963 - protein, 9 aa, synthetic construct
GGKGPDFIE

SEQ ID NO: 12964 - protein, 9 aa, synthetic construct
GGNGADVLT

SEQ ID NO: 12965 - protein, 9 aa, synthetic construct
GGSGDDIMI

SEQ ID NO: 12966 - protein, 9 aa, synthetic construct
GGFGADKLQ

SEQ ID NO: 12967 - protein, 9 aa, synthetic construct
GGSGDDILW

SEQ ID NO: 12968 - protein, 9 aa, synthetic construct
GGTGGDRLE

SEQ ID NO: 12969 - protein, 9 aa, synthetic construct
GGAGHDVLL

SEQ ID NO: 12970 - protein, 9 aa, synthetic construct
GGSGDDILQ

SEQ ID NO: 12971 - protein, 9 aa, synthetic construct
GGTGGDRLS

SEQ ID NO: 12972 - protein, 9 aa, synthetic construct
GGNGRDVLN

SEQ ID NO: 12973 - protein, 9 aa, synthetic construct
GGSGHDLIG

SEQ ID NO: 12974 - protein, 9 aa, synthetic construct
GGTGADVMV

SEQ ID NO: 12975 - protein, 9 aa, synthetic construct
GGDGYDVLY

SEQ ID NO: 12976 - protein, 9 aa, synthetic construct
GGGGDDYLS

SEQ ID NO: 12977 - protein, 9 aa, synthetic construct
GGEGNDLAA

SEQ ID NO: 12978 - protein, 9 aa, synthetic construct
GGEGDDVVR

SEQ ID NO: 12979 - protein, 9 aa, synthetic construct
GGAGNDIMD

SEQ ID NO: 12980 - protein, 9 aa, synthetic construct
GGGGNDVYF

SEQ ID NO: 12981 - protein, 9 aa, synthetic construct
GGKGNDYIS

SEQ ID NO: 12982 - protein, 9 aa, synthetic construct
GGKGNDYIV

SEQ ID NO: 12983 - protein, 9 aa, synthetic construct
GGTGADYID

SEQ ID NO: 12984 - protein, 9 aa, synthetic construct
GGAGNDIMA

SEQ ID NO: 12985 - protein, 9 aa, synthetic construct
GGAGHDVIN

SEQ ID NO: 12986 - protein, 9 aa, synthetic construct
GGIGNDQLV

SEQ ID NO: 12987 - protein, 9 aa, synthetic construct
GGDGFDTFA

SEQ ID NO: 12988 - protein, 9 aa, synthetic construct
GGEGNDLAF

SEQ ID NO: 12989 - protein, 9 aa, synthetic construct
GGKGNDVMK

SEQ ID NO: 12990 - protein, 9 aa, synthetic construct
GGFGADKLT

SEQ ID NO: 12991 - protein, 9 aa, synthetic construct
GGDGDDRIW

SEQ ID NO: 12992 - protein, 9 aa, synthetic construct
GGKGNDYLM

SEQ ID NO: 12993 - protein, 9 aa, synthetic construct
GGAGGDVLY

SEQ ID NO: 12994 - protein, 9 aa, synthetic construct
GGTGEDTLD

SEQ ID NO: 12995 - protein, 9 aa, synthetic construct
GGNGNDRMA

SEQ ID NO: 12996 - protein, 9 aa, synthetic construct
GGAGGDLIF

SEQ ID NO: 12997 - protein, 9 aa, synthetic construct
GGSGADWLS

SEQ ID NO: 12998 - protein, 9 aa, synthetic construct
GGDGDDIVY

SEQ ID NO: 12999 - protein, 9 aa, synthetic construct
GGFGADTII

SEQ ID NO: 13000 - protein, 9 aa, synthetic construct
GGSGDDSIM

SEQ ID NO: 13001 - protein, 9 aa, synthetic construct
GGSGDDSIN

SEQ ID NO: 13002 - protein, 9 aa, synthetic construct
GGSGADYID

SEQ ID NO: 13003 - protein, 9 aa, synthetic construct
GGAGNDTFD

SEQ ID NO: 13004 - protein, 9 aa, synthetic construct
GGTGHDVIQ

SEQ ID NO: 13005 - protein, 9 aa, synthetic construct
GGEGADAMT

SEQ ID NO: 13006 - protein, 9 aa, synthetic construct
GGAGGDMLT

SEQ ID NO: 13007 - protein, 9 aa, synthetic construct
GGAGADGLI

SEQ ID NO: 13008 - protein, 9 aa, synthetic construct
GGYGNDMLN

SEQ ID NO: 13009 - protein, 9 aa, synthetic construct
GGDGNDRAY

SEQ ID NO: 13010 - protein, 9 aa, synthetic construct
GGSGADWLD

SEQ ID NO: 13011 - protein, 9 aa, synthetic construct
GGIGNDTIH

SEQ ID NO: 13012 - protein, 9 aa, synthetic construct
GGIGNDTII

SEQ ID NO: 13013 - protein, 9 aa, synthetic construct
GGDGNDLVC

SEQ ID NO: 13014 - protein, 9 aa, synthetic construct
GGLGNDSIE

SEQ ID NO: 13015 - protein, 9 aa, synthetic construct
GGDGRDLLT

SEQ ID NO: 13016 - protein, 9 aa, synthetic construct
GGNGRDLLD

SEQ ID NO: 13017 - protein, 9 aa, synthetic construct
GGDGGDFVN

SEQ ID NO: 13018 - protein, 9 aa, synthetic construct
GGAGNDQVY

SEQ ID NO: 13019 - protein, 9 aa, synthetic construct
GGAGNDTAQ

SEQ ID NO: 13020 - protein, 9 aa, synthetic construct
GGTGADTLW

SEQ ID NO: 13021 - protein, 9 aa, synthetic construct
GGTGDDAID

SEQ ID NO: 13022 - protein, 9 aa, synthetic construct
GGTGHDTLQ

SEQ ID NO: 13023 - protein, 9 aa, synthetic construct
GGAGNDRAH

SEQ ID NO: 13024 - protein, 9 aa, synthetic construct
GGNGSDVII

SEQ ID NO: 13025 - protein, 9 aa, synthetic construct
GGTGHDTLS

SEQ ID NO: 13026 - protein, 9 aa, synthetic construct
GGEGDDMLS

SEQ ID NO: 13027 - protein, 9 aa, synthetic construct
GGDGDDRIA

SEQ ID NO: 13028 - protein, 9 aa, synthetic construct
GGAGLDILT

SEQ ID NO: 13029 - protein, 9 aa, synthetic construct
GGGGHDVLV

SEQ ID NO: 13030 - protein, 9 aa, synthetic construct
GGNGSDVIY

SEQ ID NO: 13031 - protein, 9 aa, synthetic construct
GGGGEDKLF

SEQ ID NO: 13032 - protein, 9 aa, synthetic construct
GGLGNDSIT

SEQ ID NO: 13033 - protein, 9 aa, synthetic construct
GGEGIDLAD

SEQ ID NO: 13034 - protein, 9 aa, synthetic construct
GGAGGDNLI

SEQ ID NO: 13035 - protein, 9 aa, synthetic construct
GGDGNDRIH

SEQ ID NO: 13036 - protein, 9 aa, synthetic construct
GGSGDDSFT

SEQ ID NO: 13037 - protein, 9 aa, synthetic construct
GGIGNDTIN

SEQ ID NO: 13038 - protein, 9 aa, synthetic construct
GGAGNDIFM

SEQ ID NO: 13039 - protein, 9 aa, synthetic construct
GGAGHDFLD

SEQ ID NO: 13040 - protein, 9 aa, synthetic construct
GGNGADTYF

SEQ ID NO: 13041 - protein, 9 aa, synthetic construct
GGDGADIMN

SEQ ID NO: 13042 - protein, 9 aa, synthetic construct
GGSGADVLK

SEQ ID NO: 13043 - protein, 9 aa, synthetic construct
GGNGADTVY

SEQ ID NO: 13044 - protein, 9 aa, synthetic construct
GGFGLDTLY

SEQ ID NO: 13045 - protein, 9 aa, synthetic construct
GGDGDDILM

SEQ ID NO: 13046 - protein, 9 aa, synthetic construct
GGSGADVLF

SEQ ID NO: 13047 - protein, 9 aa, synthetic construct
GGGGDDWLI

SEQ ID NO: 13048 - protein, 9 aa, synthetic construct
GGTGDDYLW

SEQ ID NO: 13049 - protein, 9 aa, synthetic construct
GGFGNDEIN

SEQ ID NO: 13050 - protein, 9 aa, synthetic construct
GGLGNDTYT

SEQ ID NO: 13051 - protein, 9 aa, synthetic construct
GGSGDDSVS

SEQ ID NO: 13052 - protein, 9 aa, synthetic construct
GGGGSDTMS

SEQ ID NO: 13053 - protein, 9 aa, synthetic construct
GGTGADTFT

SEQ ID NO: 13054 - protein, 9 aa, synthetic construct
GGAGHDHVN

SEQ ID NO: 13055 - protein, 9 aa, synthetic construct
GGEGADTIV

SEQ ID NO: 13056 - protein, 9 aa, synthetic construct
GGDGQDTLY

SEQ ID NO: 13057 - protein, 9 aa, synthetic construct
GGDGNDLMH

SEQ ID NO: 13058 - protein, 9 aa, synthetic construct
GGSGGDVLL

SEQ ID NO: 13059 - protein, 9 aa, synthetic construct
GGTGADTIS

SEQ ID NO: 13060 - protein, 9 aa, synthetic construct
GGNGDDYAE

SEQ ID NO: 13061 - protein, 9 aa, synthetic construct
GGDGHDILT

SEQ ID NO: 13062 - protein, 9 aa, synthetic construct
GGSGGDVLW

SEQ ID NO: 13063 - protein, 9 aa, synthetic construct
GGLGNDSIA

SEQ ID NO: 13064 - protein, 9 aa, synthetic construct
GGIGNDTIR

SEQ ID NO: 13065 - protein, 9 aa, synthetic construct
GGTGADTLG

SEQ ID NO: 13066 - protein, 9 aa, synthetic construct
GGKGNDHLD

SEQ ID NO: 13067 - protein, 9 aa, synthetic construct
GGAGGDLLW

SEQ ID NO: 13068 - protein, 9 aa, synthetic construct
GGDGHDLIY

SEQ ID NO: 13069 - protein, 9 aa, synthetic construct
GGEGADDFI

SEQ ID NO: 13070 - protein, 9 aa, synthetic construct
GGDGHDLLA

SEQ ID NO: 13071 - protein, 9 aa, synthetic construct
GGGGGDKLW

SEQ ID NO: 13072 - protein, 9 aa, synthetic construct
GGSGADVMF

SEQ ID NO: 13073 - protein, 9 aa, synthetic construct
GGYGDDVLN

SEQ ID NO: 13074 - protein, 9 aa, synthetic construct
GGGGSDKLF

SEQ ID NO: 13075 - protein, 9 aa, synthetic construct
GGAGADFLT

SEQ ID NO: 13076 - protein, 9 aa, synthetic construct
GGTGIDEMI

SEQ ID NO: 13077 - protein, 9 aa, synthetic construct
GGAGGDLLQ

SEQ ID NO: 13078 - protein, 9 aa, synthetic construct
GGGGTDLFR

SEQ ID NO: 13079 - protein, 9 aa, synthetic construct
GGDGNDLVI

SEQ ID NO: 13080 - protein, 9 aa, synthetic construct
GGDGADKLL

SEQ ID NO: 13081 - protein, 9 aa, synthetic construct
GGSGDDRVV

SEQ ID NO: 13082 - protein, 9 aa, synthetic construct
GGAGGDRFL

SEQ ID NO: 13083 - protein, 9 aa, synthetic construct
GGNGSDTID

SEQ ID NO: 13084 - protein, 9 aa, synthetic construct
GGKGDDRMM

SEQ ID NO: 13085 - protein, 9 aa, synthetic construct
GGNGADVFE

SEQ ID NO: 13086 - protein, 9 aa, synthetic construct
GGTGEDTFV

SEQ ID NO: 13087 - protein, 9 aa, synthetic construct
GGSGKDFLD

SEQ ID NO: 13088 - protein, 9 aa, synthetic construct
GGNGDDFLW

SEQ ID NO: 13089 - protein, 9 aa, synthetic construct
GGNGRDRLD

SEQ ID NO: 13090 - protein, 9 aa, synthetic construct
GGDGGDIYY

SEQ ID NO: 13091 - protein, 9 aa, synthetic construct
GGAGADIMS

SEQ ID NO: 13092 - protein, 9 aa, synthetic construct
GGLGSDVFR

SEQ ID NO: 13093 - protein, 9 aa, synthetic construct
GGSGDDDLS

SEQ ID NO: 13094 - protein, 9 aa, synthetic construct
GGSGDDDLR

SEQ ID NO: 13095 - protein, 9 aa, synthetic construct
GGDGNDLYI

SEQ ID NO: 13096 - protein, 9 aa, synthetic construct
GGTGADTMM

SEQ ID NO: 13097 - protein, 9 aa, synthetic construct
GGAGHDALA

SEQ ID NO: 13098 - protein, 9 aa, synthetic construct
GGSGDDDLE

SEQ ID NO: 13099 - protein, 9 aa, synthetic construct
GGDGADLFL

SEQ ID NO: 13100 - protein, 9 aa, synthetic construct
GGAGADIMQ

SEQ ID NO: 13101 - protein, 9 aa, synthetic construct
GGDGDDIVF

SEQ ID NO: 13102 - protein, 9 aa, synthetic construct
GGKGNDELH

SEQ ID NO: 13103 - protein, 9 aa, synthetic construct
GGGGEDIIN

SEQ ID NO: 13104 - protein, 9 aa, synthetic construct
GGAGGDYMD

SEQ ID NO: 13105 - protein, 9 aa, synthetic construct
GGAGGDYMH

SEQ ID NO: 13106 - protein, 9 aa, synthetic construct
GGDGNDVLW

SEQ ID NO: 13107 - protein, 9 aa, synthetic construct
GGDGRDSLH

SEQ ID NO: 13108 - protein, 9 aa, synthetic construct
GGAGHDVMV

SEQ ID NO: 13109 - protein, 9 aa, synthetic construct
GGSGDDELK

SEQ ID NO: 13110 - protein, 9 aa, synthetic construct
GGDGNDMIE

SEQ ID NO: 13111 - protein, 9 aa, synthetic construct
GGGGSDIYV

SEQ ID NO: 13112 - protein, 9 aa, synthetic construct
GGSGDDELF

SEQ ID NO: 13113 - protein, 9 aa, synthetic construct
GGYGFDRLN

SEQ ID NO: 13114 - protein, 9 aa, synthetic construct
GGSGDDELA

SEQ ID NO: 13115 - protein, 9 aa, synthetic construct
GGNGSDTAV

SEQ ID NO: 13116 - protein, 9 aa, synthetic construct
GGSGHDRLF

SEQ ID NO: 13117 - protein, 9 aa, synthetic construct
GGTGADTVS

SEQ ID NO: 13118 - protein, 9 aa, synthetic construct
GGNGRDRLY

SEQ ID NO: 13119 - protein, 9 aa, synthetic construct
GGNGDDRVT

SEQ ID NO: 13120 - protein, 9 aa, synthetic construct
GGIGNDLID

SEQ ID NO: 13121 - protein, 9 aa, synthetic construct
GGAGADIMV

SEQ ID NO: 13122 - protein, 9 aa, synthetic construct
GGSGDDDIT

SEQ ID NO: 13123 - protein, 9 aa, synthetic construct
GGTGDDAFI

SEQ ID NO: 13124 - protein, 9 aa, synthetic construct
GGGGNDMIF

SEQ ID NO: 13125 - protein, 9 aa, synthetic construct
GGTGADTMF

SEQ ID NO: 13126 - protein, 9 aa, synthetic construct
GGGGDDYIL

SEQ ID NO: 13127 - protein, 9 aa, synthetic construct
GGSGDDAMS

SEQ ID NO: 13128 - protein, 9 aa, synthetic construct
GGDGRDSLS

SEQ ID NO: 13129 - protein, 9 aa, synthetic construct
GGSGDDAMA

SEQ ID NO: 13130 - protein, 9 aa, synthetic construct
GGSGRDTID

SEQ ID NO: 13131 - protein, 9 aa, synthetic construct
GGIGNDIYY

SEQ ID NO: 13132 - protein, 9 aa, synthetic construct
GGLGNDSLG

SEQ ID NO: 13133 - protein, 9 aa, synthetic construct
GGKGNDEIY

SEQ ID NO: 13134 - protein, 9 aa, synthetic construct
GGAGKDTFM

SEQ ID NO: 13135 - protein, 9 aa, synthetic construct
GGEGDDTMS

SEQ ID NO: 13136 - protein, 9 aa, synthetic construct
GGEGNDLLH

SEQ ID NO: 13137 - protein, 9 aa, synthetic construct
GGSGHDSIS

SEQ ID NO: 13138 - protein, 9 aa, synthetic construct
GGIGNDIYF

SEQ ID NO: 13139 - protein, 9 aa, synthetic construct
GGAGNDIYK

SEQ ID NO: 13140 - protein, 9 aa, synthetic construct
GGNGSDTYY

SEQ ID NO: 13141 - protein, 9 aa, synthetic construct
GGEGDDWLI

SEQ ID NO: 13142 - protein, 9 aa, synthetic construct
GGYGEDRLA

SEQ ID NO: 13143 - protein, 9 aa, synthetic construct
GGTGADTMK

SEQ ID NO: 13144 - protein, 9 aa, synthetic construct
GGDGADLFI

SEQ ID NO: 13145 - protein, 9 aa, synthetic construct
GGAGLDILR

SEQ ID NO: 13146 - protein, 9 aa, synthetic construct
GGIGNDKLD

SEQ ID NO: 13147 - protein, 9 aa, synthetic construct
GGGGGDRLY

SEQ ID NO: 13148 - protein, 9 aa, synthetic construct
GGAGADIVD

SEQ ID NO: 13149 - protein, 9 aa, synthetic construct
GGAGGDQLL

SEQ ID NO: 13150 - protein, 9 aa, synthetic construct
GGFGADSVS

SEQ ID NO: 13151 - protein, 9 aa, synthetic construct
GGEGNDLIY

SEQ ID NO: 13152 - protein, 9 aa, synthetic construct
GGDGNDLVT

SEQ ID NO: 13153 - protein, 9 aa, synthetic construct
GGYGNDLLE

SEQ ID NO: 13154 - protein, 9 aa, synthetic construct
GGFGADTFA

SEQ ID NO: 13155 - protein, 9 aa, synthetic construct
GGDGNDLVS

SEQ ID NO: 13156 - protein, 9 aa, synthetic construct
GGTGEDQID

SEQ ID NO: 13157 - protein, 9 aa, synthetic construct
GGLGNDTVL

SEQ ID NO: 13158 - protein, 9 aa, synthetic construct
GGEGNDKIY

SEQ ID NO: 13159 - protein, 9 aa, synthetic construct
GGGGIDDYY

SEQ ID NO: 13160 - protein, 9 aa, synthetic construct
GGDGNDRIG

SEQ ID NO: 13161 - protein, 9 aa, synthetic construct
GGNGRDQLN

SEQ ID NO: 13162 - protein, 9 aa, synthetic construct
GGYGEDRLF

SEQ ID NO: 13163 - protein, 9 aa, synthetic construct
GGAGFDTIH

SEQ ID NO: 13164 - protein, 9 aa, synthetic construct
GGAGNDIMM

SEQ ID NO: 13165 - protein, 9 aa, synthetic construct
GGTGADNLD

SEQ ID NO: 13166 - protein, 9 aa, synthetic construct
GGEGHDVLH

SEQ ID NO: 13167 - protein, 9 aa, synthetic construct
GGAGNDKYY

SEQ ID NO: 13168 - protein, 9 aa, synthetic construct
GGLGSDIYF

SEQ ID NO: 13169 - protein, 9 aa, synthetic construct
GGSGIDVLN

SEQ ID NO: 13170 - protein, 9 aa, synthetic construct
GGCGDDALT

SEQ ID NO: 13171 - protein, 9 aa, synthetic construct
GGNGDDHLE

SEQ ID NO: 13172 - protein, 9 aa, synthetic construct
GGAGADQIF

SEQ ID NO: 13173 - protein, 9 aa, synthetic construct
GGDGNDKIY

SEQ ID NO: 13174 - protein, 9 aa, synthetic construct
GGSGEDTID

SEQ ID NO: 13175 - protein, 9 aa, synthetic construct
GGAGNDGFY

SEQ ID NO: 13176 - protein, 9 aa, synthetic construct
GGNGNDTIT

SEQ ID NO: 13177 - protein, 9 aa, synthetic construct
GGNGNDTIS

SEQ ID NO: 13178 - protein, 9 aa, synthetic construct
GGSGADALT

SEQ ID NO: 13179 - protein, 9 aa, synthetic construct
GGGGKDLLF

SEQ ID NO: 13180 - protein, 9 aa, synthetic construct
GGGGDDTMT

SEQ ID NO: 13181 - protein, 9 aa, synthetic construct
GGNGNDTIQ

SEQ ID NO: 13182 - protein, 9 aa, synthetic construct
GGKGNDQLY

SEQ ID NO: 13183 - protein, 9 aa, synthetic construct
GGAGNDKYK

SEQ ID NO: 13184 - protein, 9 aa, synthetic construct
GGYGTDTVF

SEQ ID NO: 13185 - protein, 9 aa, synthetic construct
GGAGNDFMD

SEQ ID NO: 13186 - protein, 9 aa, synthetic construct
GGSGRDRLA

SEQ ID NO: 13187 - protein, 9 aa, synthetic construct
GGDGGDLYR

SEQ ID NO: 13188 - protein, 9 aa, synthetic construct
GGGGDDTMV

SEQ ID NO: 13189 - protein, 9 aa, synthetic construct
GGDGNDRMT

SEQ ID NO: 13190 - protein, 9 aa, synthetic construct
GGAGNDMLM

SEQ ID NO: 13191 - protein, 9 aa, synthetic construct
GGDGNDKLE

SEQ ID NO: 13192 - protein, 9 aa, synthetic construct
GGAGADALH

SEQ ID NO: 13193 - protein, 9 aa, synthetic construct
GGEGADSMA

SEQ ID NO: 13194 - protein, 9 aa, synthetic construct
GGSGNDYLL

SEQ ID NO: 13195 - protein, 9 aa, synthetic construct
GGKGNDQLT

SEQ ID NO: 13196 - protein, 9 aa, synthetic construct
GGGGNDNLY

SEQ ID NO: 13197 - protein, 9 aa, synthetic construct
GGRGSDTLH

SEQ ID NO: 13198 - protein, 9 aa, synthetic construct
GGGGGDFID

SEQ ID NO: 13199 - protein, 9 aa, synthetic construct
GGPGADTLA

SEQ ID NO: 13200 - protein, 9 aa, synthetic construct
GGEGNDQLT

SEQ ID NO: 13201 - protein, 9 aa, synthetic construct
GGIGSDTLE

SEQ ID NO: 13202 - protein, 9 aa, synthetic construct
GGSGEDTVL

SEQ ID NO: 13203 - protein, 9 aa, synthetic construct
GGAGADAMD

SEQ ID NO: 13204 - protein, 9 aa, synthetic construct
GGSGIDTFV

SEQ ID NO: 13205 - protein, 9 aa, synthetic construct
GGKGSDWLD

SEQ ID NO: 13206 - protein, 9 aa, synthetic construct
GGYGSDRLS

SEQ ID NO: 13207 - protein, 9 aa, synthetic construct
GGDGFDRLD

SEQ ID NO: 13208 - protein, 9 aa, synthetic construct
GGLGNDLMH

SEQ ID NO: 13209 - protein, 9 aa, synthetic construct
GGGGQDILI

SEQ ID NO: 13210 - protein, 9 aa, synthetic construct
GGNGNDQLA

SEQ ID NO: 13211 - protein, 9 aa, synthetic construct
GGYGADLIV

SEQ ID NO: 13212 - protein, 9 aa, synthetic construct
GGAGKDVFL

SEQ ID NO: 13213 - protein, 9 aa, synthetic construct
GGGGGDKLD

SEQ ID NO: 13214 - protein, 9 aa, synthetic construct
GGPGADTLV

SEQ ID NO: 13215 - protein, 9 aa, synthetic construct
GGNGDDVLV

SEQ ID NO: 13216 - protein, 9 aa, synthetic construct
GGEGVDRLD

SEQ ID NO: 13217 - protein, 9 aa, synthetic construct
GGAGLDRLY

SEQ ID NO: 13218 - protein, 9 aa, synthetic construct
GGSGEDTLL

SEQ ID NO: 13219 - protein, 9 aa, synthetic construct
GGDGYDFLA

SEQ ID NO: 13220 - protein, 9 aa, synthetic construct
GGYGSDRIF

SEQ ID NO: 13221 - protein, 9 aa, synthetic construct
GGAGFDILL

SEQ ID NO: 13222 - protein, 9 aa, synthetic construct
GGGGNDVFY

SEQ ID NO: 13223 - protein, 9 aa, synthetic construct
GGEGVDRLF

SEQ ID NO: 13224 - protein, 9 aa, synthetic construct
GGRGSDTLS

SEQ ID NO: 13225 - protein, 9 aa, synthetic construct
GGYGTDTAS

SEQ ID NO: 13226 - protein, 9 aa, synthetic construct
GGSGRDILY

SEQ ID NO: 13227 - protein, 9 aa, synthetic construct
GGAGFDILI

SEQ ID NO: 13228 - protein, 9 aa, synthetic construct
GGMGADTAI

SEQ ID NO: 13229 - protein, 9 aa, synthetic construct
GGAGNDFMN

SEQ ID NO: 13230 - protein, 9 aa, synthetic construct
GGKGKDTFI

SEQ ID NO: 13231 - protein, 9 aa, synthetic construct
GGEGRDRLD

SEQ ID NO: 13232 - protein, 9 aa, synthetic construct
GGSGEDVFV

SEQ ID NO: 13233 - protein, 9 aa, synthetic construct
GGLGNDMLI

SEQ ID NO: 13234 - protein, 9 aa, synthetic construct
GGIGNDYLF

SEQ ID NO: 13235 - protein, 9 aa, synthetic construct
GGFGTDTLF

SEQ ID NO: 13236 - protein, 9 aa, synthetic construct
GGEGDDRLQ

SEQ ID NO: 13237 - protein, 9 aa, synthetic construct
GGEGNDQLL

SEQ ID NO: 13238 - protein, 9 aa, synthetic construct
GGIGSDTIS

SEQ ID NO: 13239 - protein, 9 aa, synthetic construct
GGDGSDILT

SEQ ID NO: 13240 - protein, 9 aa, synthetic construct
GGGGDDTVR

SEQ ID NO: 13241 - protein, 9 aa, synthetic construct
GGTGDDNLN

SEQ ID NO: 13242 - protein, 9 aa, synthetic construct
GGDGEDLIY

SEQ ID NO: 13243 - protein, 9 aa, synthetic construct
GGEGADYLS

SEQ ID NO: 13244 - protein, 9 aa, synthetic construct
GGSGEDRLH

SEQ ID NO: 13245 - protein, 9 aa, synthetic construct
GGDGEDTYV

SEQ ID NO: 13246 - protein, 9 aa, synthetic construct
GGNGNDQLK

SEQ ID NO: 13247 - protein, 9 aa, synthetic construct
GGAGKDWLD

SEQ ID NO: 13248 - protein, 9 aa, synthetic construct
GGWGSDILQ

SEQ ID NO: 13249 - protein, 9 aa, synthetic construct
GGMGADRLG

SEQ ID NO: 13250 - protein, 9 aa, synthetic construct
GGDGNDILK

SEQ ID NO: 13251 - protein, 9 aa, synthetic construct
GGGGTDTLS

SEQ ID NO: 13252 - protein, 9 aa, synthetic construct
GGGGHDWLS

SEQ ID NO: 13253 - protein, 9 aa, synthetic construct
GGTGNDLIN

SEQ ID NO: 13254 - protein, 9 aa, synthetic construct
GGTGNDELF

SEQ ID NO: 13255 - protein, 9 aa, synthetic construct
GGAGNDVYR

SEQ ID NO: 13256 - protein, 9 aa, synthetic construct
GGTGNDEIW

SEQ ID NO: 13257 - protein, 9 aa, synthetic construct
GGIGNDYLD

SEQ ID NO: 13258 - protein, 9 aa, synthetic construct
GGPGADRLE

SEQ ID NO: 13259 - protein, 9 aa, synthetic construct
GGLGSDTMI

SEQ ID NO: 13260 - protein, 9 aa, synthetic construct
GGAGNDVYH

SEQ ID NO: 13261 - protein, 9 aa, synthetic construct
GGFGRDVLF

SEQ ID NO: 13262 - protein, 9 aa, synthetic construct
GGFGRDVLI

SEQ ID NO: 13263 - protein, 9 aa, synthetic construct
GGCGNDRIV

SEQ ID NO: 13264 - protein, 9 aa, synthetic construct
GGKGSDRFV

SEQ ID NO: 13265 - protein, 9 aa, synthetic construct
GGSGFDTLG

SEQ ID NO: 13266 - protein, 9 aa, synthetic construct
GGNGNDNLQ

SEQ ID NO: 13267 - protein, 9 aa, synthetic construct
GGRGSDSLI

SEQ ID NO: 13268 - protein, 9 aa, synthetic construct
GGDGHDRLL

SEQ ID NO: 13269 - protein, 9 aa, synthetic construct
GGFGVDTIV

SEQ ID NO: 13270 - protein, 9 aa, synthetic construct
GGTGNDFLR

SEQ ID NO: 13271 - protein, 9 aa, synthetic construct
GGGGDDTVD

SEQ ID NO: 13272 - protein, 9 aa, synthetic construct
GGEGNDYIS

SEQ ID NO: 13273 - protein, 9 aa, synthetic construct
GGEGHDVIN

SEQ ID NO: 13274 - protein, 9 aa, synthetic construct
GGAGADDLN

SEQ ID NO: 13275 - protein, 9 aa, synthetic construct
GGGGSDSIL

SEQ ID NO: 13276 - protein, 9 aa, synthetic construct
GGEGADEME

SEQ ID NO: 13277 - protein, 9 aa, synthetic construct
GGAGLDRLS

SEQ ID NO: 13278 - protein, 9 aa, synthetic construct
GGGGGDYIQ

SEQ ID NO: 13279 - protein, 9 aa, synthetic construct
GGGGNDNLS

SEQ ID NO: 13280 - protein, 9 aa, synthetic construct
GGTGADQLF

SEQ ID NO: 13281 - protein, 9 aa, synthetic construct
GGEGIDTLY

SEQ ID NO: 13282 - protein, 9 aa, synthetic construct
GGSGNDYLI

SEQ ID NO: 13283 - protein, 9 aa, synthetic construct
GGTGDDNLD

SEQ ID NO: 13284 - protein, 9 aa, synthetic construct
GGTGNDFLF

SEQ ID NO: 13285 - protein, 9 aa, synthetic construct
GGAGADMIY

SEQ ID NO: 13286 - protein, 9 aa, synthetic construct
GGLGNDLIT

SEQ ID NO: 13287 - protein, 9 aa, synthetic construct
GGNGADRLT

SEQ ID NO: 13288 - protein, 9 aa, synthetic construct
GGAGNDLMG

SEQ ID NO: 13289 - protein, 9 aa, synthetic construct
GGAGADDLV

SEQ ID NO: 13290 - protein, 9 aa, synthetic construct
GGLGNDLYV

SEQ ID NO: 13291 - protein, 9 aa, synthetic construct
GGTGNDLIA

SEQ ID NO: 13292 - protein, 9 aa, synthetic construct
GGNGNDQLH

SEQ ID NO: 13293 - protein, 9 aa, synthetic construct
GGFGNDVLT

SEQ ID NO: 13294 - protein, 9 aa, synthetic construct
GGAGNDWIA

SEQ ID NO: 13295 - protein, 9 aa, synthetic construct
GGSGRDILI

SEQ ID NO: 13296 - protein, 9 aa, synthetic construct
GGNGEDILI

SEQ ID NO: 13297 - protein, 9 aa, synthetic construct
GGKGNDNLY

SEQ ID NO: 13298 - protein, 9 aa, synthetic construct
GGSGEDVID

SEQ ID NO: 13299 - protein, 9 aa, synthetic construct
GGNGDDYLN

SEQ ID NO: 13300 - protein, 9 aa, synthetic construct
GGAGKDRLV

SEQ ID NO: 13301 - protein, 9 aa, synthetic construct
GGNGNDTMD

SEQ ID NO: 13302 - protein, 9 aa, synthetic construct
GGDGEDSLL

SEQ ID NO: 13303 - protein, 9 aa, synthetic construct
GGEGNDYLI

SEQ ID NO: 13304 - protein, 9 aa, synthetic construct
GGDGHDEMY

SEQ ID NO: 13305 - protein, 9 aa, synthetic construct
GGDGRDILT

SEQ ID NO: 13306 - protein, 9 aa, synthetic construct
GGTGDDFMV

SEQ ID NO: 13307 - protein, 9 aa, synthetic construct
GGWGYDTLD

SEQ ID NO: 13308 - protein, 9 aa, synthetic construct
GGTGNDKAW

SEQ ID NO: 13309 - protein, 9 aa, synthetic construct
GGFGRDSLD

SEQ ID NO: 13310 - protein, 9 aa, synthetic construct
GGAGKDVLV

SEQ ID NO: 13311 - protein, 9 aa, synthetic construct
GGTGNDIIK

SEQ ID NO: 13312 - protein, 9 aa, synthetic construct
GGAGNDYIN

SEQ ID NO: 13313 - protein, 9 aa, synthetic construct
GGNGDDHLH

SEQ ID NO: 13314 - protein, 9 aa, synthetic construct
GGNGNDTVN

SEQ ID NO: 13315 - protein, 9 aa, synthetic construct
GGNGDDSII

SEQ ID NO: 13316 - protein, 9 aa, synthetic construct
GGAGNDLVI

SEQ ID NO: 13317 - protein, 9 aa, synthetic construct
GGMGDDTLL

SEQ ID NO: 13318 - protein, 9 aa, synthetic construct
GGGGNDLLW

SEQ ID NO: 13319 - protein, 9 aa, synthetic construct
GGNGDDRLA

SEQ ID NO: 13320 - protein, 9 aa, synthetic construct
GGPGADWLD

SEQ ID NO: 13321 - protein, 9 aa, synthetic construct
GGAGHDRIA

SEQ ID NO: 13322 - protein, 9 aa, synthetic construct
GGAGNDYIH

SEQ ID NO: 13323 - protein, 9 aa, synthetic construct
GGTGDDLII

SEQ ID NO: 13324 - protein, 9 aa, synthetic construct
GGDGDDKLV

SEQ ID NO: 13325 - protein, 9 aa, synthetic construct
GGAGNDLFI

SEQ ID NO: 13326 - protein, 9 aa, synthetic construct
GGAGNDYVD

SEQ ID NO: 13327 - protein, 9 aa, synthetic construct
GGAGADNLQ

SEQ ID NO: 13328 - protein, 9 aa, synthetic construct
GGKGKDTLK

SEQ ID NO: 13329 - protein, 9 aa, synthetic construct
GGNGNDTYE

SEQ ID NO: 13330 - protein, 9 aa, synthetic construct
GGKGSDTMS

SEQ ID NO: 13331 - protein, 9 aa, synthetic construct
GGLGTDKLI

SEQ ID NO: 13332 - protein, 9 aa, synthetic construct
GGDGNDIVQ

SEQ ID NO: 13333 - protein, 9 aa, synthetic construct
GGNGDDSLA

SEQ ID NO: 13334 - protein, 9 aa, synthetic construct
GGWGSDVLT

SEQ ID NO: 13335 - protein, 9 aa, synthetic construct
GGDGDDKLN

SEQ ID NO: 13336 - protein, 9 aa, synthetic construct
GGNGADQMY

SEQ ID NO: 13337 - protein, 9 aa, synthetic construct
GGAGYDTLL

SEQ ID NO: 13338 - protein, 9 aa, synthetic construct
GGDGNDVIA

SEQ ID NO: 13339 - protein, 9 aa, synthetic construct
GGEGRDRFE

SEQ ID NO: 13340 - protein, 9 aa, synthetic construct
GGTGNDIMR

SEQ ID NO: 13341 - protein, 9 aa, synthetic construct
GGSGGDILT

SEQ ID NO: 13342 - protein, 9 aa, synthetic construct
GGTGNDIVN

SEQ ID NO: 13343 - protein, 9 aa, synthetic construct
GGKGKDTLT

SEQ ID NO: 13344 - protein, 9 aa, synthetic construct
GGAGNDYLT

SEQ ID NO: 13345 - protein, 9 aa, synthetic construct
GGDGEDSLI

SEQ ID NO: 13346 - protein, 9 aa, synthetic construct
GGWGSDYLR

SEQ ID NO: 13347 - protein, 9 aa, synthetic construct
GGSGSDHLE

SEQ ID NO: 13348 - protein, 9 aa, synthetic construct
GGTGDDLLN

SEQ ID NO: 13349 - protein, 9 aa, synthetic construct
GGTGDDLIS

SEQ ID NO: 13350 - protein, 9 aa, synthetic construct
GGAGKDVMA

SEQ ID NO: 13351 - protein, 9 aa, synthetic construct
GGAGNDLYL

SEQ ID NO: 13352 - protein, 9 aa, synthetic construct
GGDGWDTLY

SEQ ID NO: 13353 - protein, 9 aa, synthetic construct
GGIGFDTLH

SEQ ID NO: 13354 - protein, 9 aa, synthetic construct
GGAGNDYLW

SEQ ID NO: 13355 - protein, 9 aa, synthetic construct
GGTGNDILW

SEQ ID NO: 13356 - protein, 9 aa, synthetic construct
GGTGNDIIY

SEQ ID NO: 13357 - protein, 9 aa, synthetic construct
GGAGHDTAR

SEQ ID NO: 13358 - protein, 9 aa, synthetic construct
GGTGADNMT

SEQ ID NO: 13359 - protein, 9 aa, synthetic construct
GGAGNDLVV

SEQ ID NO: 13360 - protein, 9 aa, synthetic construct
GGSGFDEVS

SEQ ID NO: 13361 - protein, 9 aa, synthetic construct
GGAGNDYMD

SEQ ID NO: 13362 - protein, 9 aa, synthetic construct
GGTGNDIIR

SEQ ID NO: 13363 - protein, 9 aa, synthetic construct
GGYGSDTLD

SEQ ID NO: 13364 - protein, 9 aa, synthetic construct
GGDGEDSLN

SEQ ID NO: 13365 - protein, 9 aa, synthetic construct
GGTGNDIFY

SEQ ID NO: 13366 - protein, 9 aa, synthetic construct
GGDGADVIL

SEQ ID NO: 13367 - protein, 9 aa, synthetic construct
GGDGNDKIF

SEQ ID NO: 13368 - protein, 9 aa, synthetic construct
GGDGNDRVD

SEQ ID NO: 13369 - protein, 9 aa, synthetic construct
GGDGNDKID

SEQ ID NO: 13370 - protein, 9 aa, synthetic construct
GGSGRDLIY

SEQ ID NO: 13371 - protein, 9 aa, synthetic construct
GGTGADNLN

SEQ ID NO: 13372 - protein, 9 aa, synthetic construct
GGNGNDTYR

SEQ ID NO: 13373 - protein, 9 aa, synthetic construct
GGKGSDTIY

SEQ ID NO: 13374 - protein, 9 aa, synthetic construct
GGDGDDIFL

SEQ ID NO: 13375 - protein, 9 aa, synthetic construct
GGSGNDYLR

SEQ ID NO: 13376 - protein, 9 aa, synthetic construct
GGAGFDILS

SEQ ID NO: 13377 - protein, 9 aa, synthetic construct
GGAGFDILR

SEQ ID NO: 13378 - protein, 9 aa, synthetic construct
GGEGRDNYW

SEQ ID NO: 13379 - protein, 9 aa, synthetic construct
GGDGNDQIW

SEQ ID NO: 13380 - protein, 9 aa, synthetic construct
GGPGADVID

SEQ ID NO: 13381 - protein, 9 aa, synthetic construct
GGMGADTIY

SEQ ID NO: 13382 - protein, 9 aa, synthetic construct
GGGGHDILS

SEQ ID NO: 13383 - protein, 9 aa, synthetic construct
GGEGKDWIE

SEQ ID NO: 13384 - protein, 9 aa, synthetic construct
GGDGADTVL

SEQ ID NO: 13385 - protein, 9 aa, synthetic construct
GGAGNDLMY

SEQ ID NO: 13386 - protein, 9 aa, synthetic construct
GGAGNDFMY

SEQ ID NO: 13387 - protein, 9 aa, synthetic construct
GGAGNDLMW

SEQ ID NO: 13388 - protein, 9 aa, synthetic construct
GGSGFDSFF

SEQ ID NO: 13389 - protein, 9 aa, synthetic construct
GGYGADIVR

SEQ ID NO: 13390 - protein, 9 aa, synthetic construct
GGNGNDQIS

SEQ ID NO: 13391 - protein, 9 aa, synthetic construct
GGSGEDVLF

SEQ ID NO: 13392 - protein, 9 aa, synthetic construct
GGGGDDTFY

SEQ ID NO: 13393 - protein, 9 aa, synthetic construct
GGTGDDFVS

SEQ ID NO: 13394 - protein, 9 aa, synthetic construct
GGAGADMLY

SEQ ID NO: 13395 - protein, 9 aa, synthetic construct
GGAGNDWLQ

SEQ ID NO: 13396 - protein, 9 aa, synthetic construct
GGEGADFLD

SEQ ID NO: 13397 - protein, 9 aa, synthetic construct
GGRGSDTYV

SEQ ID NO: 13398 - protein, 9 aa, synthetic construct
GGEGIDTVD

SEQ ID NO: 13399 - protein, 9 aa, synthetic construct
GGDGHDFLA

SEQ ID NO: 13400 - protein, 9 aa, synthetic construct
GGNGNDTYL

SEQ ID NO: 13401 - protein, 9 aa, synthetic construct
GGMGDDTLA

SEQ ID NO: 13402 - protein, 9 aa, synthetic construct
GGPGADVMT

SEQ ID NO: 13403 - protein, 9 aa, synthetic construct
GGAGNDYFY

SEQ ID NO: 13404 - protein, 9 aa, synthetic construct
GGEGADFLN

SEQ ID NO: 13405 - protein, 9 aa, synthetic construct
GGDGDDIFI

SEQ ID NO: 13406 - protein, 9 aa, synthetic construct
GGNGNDSML

SEQ ID NO: 13407 - protein, 9 aa, synthetic construct
GGSGEDYLH

SEQ ID NO: 13408 - protein, 9 aa, synthetic construct
GGFGDDELR

SEQ ID NO: 13409 - protein, 9 aa, synthetic construct
GGMGDDTLF

SEQ ID NO: 13410 - protein, 9 aa, synthetic construct
GGDGEDSLS

SEQ ID NO: 13411 - protein, 9 aa, synthetic construct
GGEGVDNLF

SEQ ID NO: 13412 - protein, 9 aa, synthetic construct
GGFGVDHLH

SEQ ID NO: 13413 - protein, 9 aa, synthetic construct
GGAGADNLF

SEQ ID NO: 13414 - protein, 9 aa, synthetic construct
GGGGQDIVD

SEQ ID NO: 13415 - protein, 9 aa, synthetic construct
GGSGIDTLK

SEQ ID NO: 13416 - protein, 9 aa, synthetic construct
GGDGNDQLE

SEQ ID NO: 13417 - protein, 9 aa, synthetic construct
GGEGNDQVL

SEQ ID NO: 13418 - protein, 9 aa, synthetic construct
GGDGNDIMV

SEQ ID NO: 13419 - protein, 9 aa, synthetic construct
GGTGDDLFV

SEQ ID NO: 13420 - protein, 9 aa, synthetic construct
GGDGNDVYL

SEQ ID NO: 13421 - protein, 9 aa, synthetic construct
GGDGNDRVV

SEQ ID NO: 13422 - protein, 9 aa, synthetic construct
GGKGSDVLR

SEQ ID NO: 13423 - protein, 9 aa, synthetic construct
GGAGNDLFL

SEQ ID NO: 13424 - protein, 9 aa, synthetic construct
GGAGNDMIF

SEQ ID NO: 13425 - protein, 9 aa, synthetic construct
GGAGADNIS

SEQ ID NO: 13426 - protein, 9 aa, synthetic construct
GGYGADAFI

SEQ ID NO: 13427 - protein, 9 aa, synthetic construct
GGAGNDWVR

SEQ ID NO: 13428 - protein, 9 aa, synthetic construct
GGAGNDYVY

SEQ ID NO: 13429 - protein, 9 aa, synthetic construct
GGRGVDTAV

SEQ ID NO: 13430 - protein, 9 aa, synthetic construct
GGSGEDVMT

SEQ ID NO: 13431 - protein, 9 aa, synthetic construct
GGKGNDLLL

SEQ ID NO: 13432 - protein, 9 aa, synthetic construct
GGNGNDTML

SEQ ID NO: 13433 - protein, 9 aa, synthetic construct
GGSGADHLN

SEQ ID NO: 13434 - protein, 9 aa, synthetic construct
GGDGSDELR

SEQ ID NO: 13435 - protein, 9 aa, synthetic construct
GGLGNDWLD

SEQ ID NO: 13436 - protein, 9 aa, synthetic construct
GGAGADEFK

SEQ ID NO: 13437 - protein, 9 aa, synthetic construct
GGNGDDRLQ

SEQ ID NO: 13438 - protein, 9 aa, synthetic construct
GGSGEDIIT

SEQ ID NO: 13439 - protein, 9 aa, synthetic construct
GGNGFDVAS

SEQ ID NO: 13440 - protein, 9 aa, synthetic construct
GGAGNDVMQ

SEQ ID NO: 13441 - protein, 9 aa, synthetic construct
GGNGDDVLK

SEQ ID NO: 13442 - protein, 9 aa, synthetic construct
GGTGNDDID

SEQ ID NO: 13443 - protein, 9 aa, synthetic construct
GGEGADVLV

SEQ ID NO: 13444 - protein, 9 aa, synthetic construct
GGAGNDNLM

SEQ ID NO: 13445 - protein, 9 aa, synthetic construct
GGDGDDSML

SEQ ID NO: 13446 - protein, 9 aa, synthetic construct
GGIGNDVYY

SEQ ID NO: 13447 - protein, 9 aa, synthetic construct
GGEGQDLLQ

SEQ ID NO: 13448 - protein, 9 aa, synthetic construct
GGTGDDIFK

SEQ ID NO: 13449 - protein, 9 aa, synthetic construct
GGAGHDLVY

SEQ ID NO: 13450 - protein, 9 aa, synthetic construct
GGNGDDYLI

SEQ ID NO: 13451 - protein, 9 aa, synthetic construct
GGNGNDWLC

SEQ ID NO: 13452 - protein, 9 aa, synthetic construct
GGWGRDTFI

SEQ ID NO: 13453 - protein, 9 aa, synthetic construct
GGSGEDFIF

SEQ ID NO: 13454 - protein, 9 aa, synthetic construct
GGKGNDRLL

SEQ ID NO: 13455 - protein, 9 aa, synthetic construct
GGTGADMLY

SEQ ID NO: 13456 - protein, 9 aa, synthetic construct
GGKGLDKLS

SEQ ID NO: 13457 - protein, 9 aa, synthetic construct
GGLGYDNLY

SEQ ID NO: 13458 - protein, 9 aa, synthetic construct
GGGGDDTYL

SEQ ID NO: 13459 - protein, 9 aa, synthetic construct
GGTGNDDLL

SEQ ID NO: 13460 - protein, 9 aa, synthetic construct
GGDGNDILC

SEQ ID NO: 13461 - protein, 9 aa, synthetic construct
GGSGADIFQ

SEQ ID NO: 13462 - protein, 9 aa, synthetic construct
GGDGNDVFS

SEQ ID NO: 13463 - protein, 9 aa, synthetic construct
GGAGHDSID

SEQ ID NO: 13464 - protein, 9 aa, synthetic construct
GGEGNDQIS

SEQ ID NO: 13465 - protein, 9 aa, synthetic construct
GGAGNDLIG

SEQ ID NO: 13466 - protein, 9 aa, synthetic construct
GGLGTDMLT

SEQ ID NO: 13467 - protein, 9 aa, synthetic construct
GGAGADQLG

SEQ ID NO: 13468 - protein, 9 aa, synthetic construct
GGMGADTLV

SEQ ID NO: 13469 - protein, 9 aa, synthetic construct
GGYGADTLN

SEQ ID NO: 13470 - protein, 9 aa, synthetic construct
GGAGNDVMV

SEQ ID NO: 13471 - protein, 9 aa, synthetic construct
GGKGDDTIR

SEQ ID NO: 13472 - protein, 9 aa, synthetic construct
GGTGDDQVF

SEQ ID NO: 13473 - protein, 9 aa, synthetic construct
GGDGRDHLS

SEQ ID NO: 13474 - protein, 9 aa, synthetic construct
GGNGNDTFY

SEQ ID NO: 13475 - protein, 9 aa, synthetic construct
GGTGDDRFF

SEQ ID NO: 13476 - protein, 9 aa, synthetic construct
GGAGNDVMI

SEQ ID NO: 13477 - protein, 9 aa, synthetic construct
GGSGADIFA

SEQ ID NO: 13478 - protein, 9 aa, synthetic construct
GGNGNDWLS

SEQ ID NO: 13479 - protein, 9 aa, synthetic construct
GGTGNDALH

SEQ ID NO: 13480 - protein, 9 aa, synthetic construct
GGSGGDAFV

SEQ ID NO: 13481 - protein, 9 aa, synthetic construct
GGGGTDTLA

SEQ ID NO: 13482 - protein, 9 aa, synthetic construct
GGDGNDYAY

SEQ ID NO: 13483 - protein, 9 aa, synthetic construct
GGRGSDLLE

SEQ ID NO: 13484 - protein, 9 aa, synthetic construct
GGEGDDLII

SEQ ID NO: 13485 - protein, 9 aa, synthetic construct
GGAGADQLE

SEQ ID NO: 13486 - protein, 9 aa, synthetic construct
GGGGPDVLR

SEQ ID NO: 13487 - protein, 9 aa, synthetic construct
GGTGNDALM

SEQ ID NO: 13488 - protein, 9 aa, synthetic construct
GGLGNDYMI

SEQ ID NO: 13489 - protein, 9 aa, synthetic construct
GGSGFDWLE

SEQ ID NO: 13490 - protein, 9 aa, synthetic construct
GGPGADKLD

SEQ ID NO: 13491 - protein, 9 aa, synthetic construct
GGTGNDLYF

SEQ ID NO: 13492 - protein, 9 aa, synthetic construct
GGDGADALN

SEQ ID NO: 13493 - protein, 9 aa, synthetic construct
GGSGADIFI

SEQ ID NO: 13494 - protein, 9 aa, synthetic construct
GGRGSDMLM

SEQ ID NO: 13495 - protein, 9 aa, synthetic construct
GGEGQDSLD

SEQ ID NO: 13496 - protein, 9 aa, synthetic construct
GGDGADALD

SEQ ID NO: 13497 - protein, 9 aa, synthetic construct
GGNGNDTAA

SEQ ID NO: 13498 - protein, 9 aa, synthetic construct
GGTGNDLVS

SEQ ID NO: 13499 - protein, 9 aa, synthetic construct
GGAGADAFF

SEQ ID NO: 13500 - protein, 9 aa, synthetic construct
GGYGADTLD

SEQ ID NO: 13501 - protein, 9 aa, synthetic construct
GGAGNDFLL

SEQ ID NO: 13502 - protein, 9 aa, synthetic construct
GGAGPDTFI

SEQ ID NO: 13503 - protein, 9 aa, synthetic construct
GGNGDDEID

SEQ ID NO: 13504 - protein, 9 aa, synthetic construct
GGDGNDSAD

SEQ ID NO: 13505 - protein, 9 aa, synthetic construct
GGYGADTLF

SEQ ID NO: 13506 - protein, 9 aa, synthetic construct
GGTGDDQLQ

SEQ ID NO: 13507 - protein, 9 aa, synthetic construct
GGIGQDTLD

SEQ ID NO: 13508 - protein, 9 aa, synthetic construct
GGNGNDWVR

SEQ ID NO: 13509 - protein, 9 aa, synthetic construct
GGTGNDLYY

SEQ ID NO: 13510 - protein, 9 aa, synthetic construct
GGFGYDFLW

SEQ ID NO: 13511 - protein, 9 aa, synthetic construct
GGAGNDGLT

SEQ ID NO: 13512 - protein, 9 aa, synthetic construct
GGPGDDIIT

SEQ ID NO: 13513 - protein, 9 aa, synthetic construct
GGTGNDDLA

SEQ ID NO: 13514 - protein, 9 aa, synthetic construct
GGKGDDAYG

SEQ ID NO: 13515 - protein, 9 aa, synthetic construct
GGAGADAFI

SEQ ID NO: 13516 - protein, 9 aa, synthetic construct
GGNGNDSLQ

SEQ ID NO: 13517 - protein, 9 aa, synthetic construct
GGTGDDILF

SEQ ID NO: 13518 - protein, 9 aa, synthetic construct
GGAGFDSLM

SEQ ID NO: 13519 - protein, 9 aa, synthetic construct
GGAGLDRLE

SEQ ID NO: 13520 - protein, 9 aa, synthetic construct
GGLGNDMLT

SEQ ID NO: 13521 - protein, 9 aa, synthetic construct
GGEGADTFK

SEQ ID NO: 13522 - protein, 9 aa, synthetic construct
GGTGADRFD

SEQ ID NO: 13523 - protein, 9 aa, synthetic construct
GGDGADDFV

SEQ ID NO: 13524 - protein, 9 aa, synthetic construct
GGEGDDVYL

SEQ ID NO: 13525 - protein, 9 aa, synthetic construct
GGSGGDALY

SEQ ID NO: 13526 - protein, 9 aa, synthetic construct
GGSGDDYVS

SEQ ID NO: 13527 - protein, 9 aa, synthetic construct
GGAGNDNMI

SEQ ID NO: 13528 - protein, 9 aa, synthetic construct
GGDGDDQLW

SEQ ID NO: 13529 - protein, 9 aa, synthetic construct
GGGGGDFLY

SEQ ID NO: 13530 - protein, 9 aa, synthetic construct
GGNGNDSLR

SEQ ID NO: 13531 - protein, 9 aa, synthetic construct
GGAGHDMLD

SEQ ID NO: 13532 - protein, 9 aa, synthetic construct
GGDGQDSLV

SEQ ID NO: 13533 - protein, 9 aa, synthetic construct
GGDGQDTFV

SEQ ID NO: 13534 - protein, 9 aa, synthetic construct
GGAGNDGLR

SEQ ID NO: 13535 - protein, 9 aa, synthetic construct
GGSGGDALR

SEQ ID NO: 13536 - protein, 9 aa, synthetic construct
GGNGDDSIT

SEQ ID NO: 13537 - protein, 9 aa, synthetic construct
GGAGHDRMF

SEQ ID NO: 13538 - protein, 9 aa, synthetic construct
GGDGNDRMD

SEQ ID NO: 13539 - protein, 9 aa, synthetic construct
GGAGLDRLF

SEQ ID NO: 13540 - protein, 9 aa, synthetic construct
GGLGNDVYY

SEQ ID NO: 13541 - protein, 9 aa, synthetic construct
GGEGVDTIY

SEQ ID NO: 13542 - protein, 9 aa, synthetic construct
GGAGNDNFV

SEQ ID NO: 13543 - protein, 9 aa, synthetic construct
GGDGADTIQ

SEQ ID NO: 13544 - protein, 9 aa, synthetic construct
GGAGNDGIT

SEQ ID NO: 13545 - protein, 9 aa, synthetic construct
GGKGDDLLA

SEQ ID NO: 13546 - protein, 9 aa, synthetic construct
GGTGMDVLF

SEQ ID NO: 13547 - protein, 9 aa, synthetic construct
GGLGNDKLL

SEQ ID NO: 13548 - protein, 9 aa, synthetic construct
GGIGSDTMT

SEQ ID NO: 13549 - protein, 9 aa, synthetic construct
GGSGADILH

SEQ ID NO: 13550 - protein, 9 aa, synthetic construct
GGRGSDRLF

SEQ ID NO: 13551 - protein, 9 aa, synthetic construct
GGFGKDSLD

SEQ ID NO: 13552 - protein, 9 aa, synthetic construct
GGAGFDTFV

SEQ ID NO: 13553 - protein, 9 aa, synthetic construct
GGEGADELI

SEQ ID NO: 13554 - protein, 9 aa, synthetic construct
GGSGGDELK

SEQ ID NO: 13555 - protein, 9 aa, synthetic construct
GGSGGDDFD

SEQ ID NO: 13556 - protein, 9 aa, synthetic construct
GGEGHDTLY

SEQ ID NO: 13557 - protein, 9 aa, synthetic construct
GGTGDDRFT

SEQ ID NO: 13558 - protein, 9 aa, synthetic construct
GGYGADTLL

SEQ ID NO: 13559 - protein, 9 aa, synthetic construct
GGDGDDKID

SEQ ID NO: 13560 - protein, 9 aa, synthetic construct
GGAGNDVVH

SEQ ID NO: 13561 - protein, 9 aa, synthetic construct
GGYGADTII

SEQ ID NO: 13562 - protein, 9 aa, synthetic construct
GGDGNDKVF

SEQ ID NO: 13563 - protein, 9 aa, synthetic construct
GGNGFDTLR

SEQ ID NO: 13564 - protein, 9 aa, synthetic construct
GGTGNDAMT

SEQ ID NO: 13565 - protein, 9 aa, synthetic construct
GGTGDDRFI

SEQ ID NO: 13566 - protein, 9 aa, synthetic construct
GGAGFDSLL

SEQ ID NO: 13567 - protein, 9 aa, synthetic construct
GGDGADAFV

SEQ ID NO: 13568 - protein, 9 aa, synthetic construct
GGTGNDLVD

SEQ ID NO: 13569 - protein, 9 aa, synthetic construct
GGFGSDEVL

SEQ ID NO: 13570 - protein, 9 aa, synthetic construct
GGPGADQID

SEQ ID NO: 13571 - protein, 9 aa, synthetic construct
GGAGNDGLF

SEQ ID NO: 13572 - protein, 9 aa, synthetic construct
GGAGFDTAV

SEQ ID NO: 13573 - protein, 9 aa, synthetic construct
GGFGDDRIS

SEQ ID NO: 13574 - protein, 9 aa, synthetic construct
GGFGTDLIE

SEQ ID NO: 13575 - protein, 9 aa, synthetic construct
GGEGDDLIK

SEQ ID NO: 13576 - protein, 9 aa, synthetic construct
GGAGFDSLI

SEQ ID NO: 13577 - protein, 9 aa, synthetic construct
GGDGDDIIH

SEQ ID NO: 13578 - protein, 9 aa, synthetic construct
GGDGADTME

SEQ ID NO: 13579 - protein, 9 aa, synthetic construct
GGDGADAFM

SEQ ID NO: 13580 - protein, 9 aa, synthetic construct
GGTGDDRFV

SEQ ID NO: 13581 - protein, 9 aa, synthetic construct
GGSGRDLLT

SEQ ID NO: 13582 - protein, 9 aa, synthetic construct
GGSGIDNLT

SEQ ID NO: 13583 - protein, 9 aa, synthetic construct
GGTGDDQIF

SEQ ID NO: 13584 - protein, 9 aa, synthetic construct
GGDGDDQLV

SEQ ID NO: 13585 - protein, 9 aa, synthetic construct
GGTGDDRIV

SEQ ID NO: 13586 - protein, 9 aa, synthetic construct
GGAGADHLR

SEQ ID NO: 13587 - protein, 9 aa, synthetic construct
GGDGDDVVI

SEQ ID NO: 13588 - protein, 9 aa, synthetic construct
GGGGDDFVF

SEQ ID NO: 13589 - protein, 9 aa, synthetic construct
GGNGNDEVI

SEQ ID NO: 13590 - protein, 9 aa, synthetic construct
GGQGDDTIV

SEQ ID NO: 13591 - protein, 9 aa, synthetic construct
GGYGNDDLN

SEQ ID NO: 13592 - protein, 9 aa, synthetic construct
GGNGNDSFV

SEQ ID NO: 13593 - protein, 9 aa, synthetic construct
GGKGFDIID

SEQ ID NO: 13594 - protein, 9 aa, synthetic construct
GGGGDDHLS

SEQ ID NO: 13595 - protein, 9 aa, synthetic construct
GGSGQDYLN

SEQ ID NO: 13596 - protein, 9 aa, synthetic construct
GGEGNDEIF

SEQ ID NO: 13597 - protein, 9 aa, synthetic construct
GGVGKDTLT

SEQ ID NO: 13598 - protein, 9 aa, synthetic construct
GGYGNDALN

SEQ ID NO: 13599 - protein, 9 aa, synthetic construct
GGAGADHLT

SEQ ID NO: 13600 - protein, 9 aa, synthetic construct
GGVGNDVFE

SEQ ID NO: 13601 - protein, 9 aa, synthetic construct
GGKGEDDLK

SEQ ID NO: 13602 - protein, 9 aa, synthetic construct
GGMGNDKLD

SEQ ID NO: 13603 - protein, 9 aa, synthetic construct
GGVGNDSLW

SEQ ID NO: 13604 - protein, 9 aa, synthetic construct
GGYGNDALE

SEQ ID NO: 13605 - protein, 9 aa, synthetic construct
GGSGTDTLA

SEQ ID NO: 13606 - protein, 9 aa, synthetic construct
GGVGIDTMI

SEQ ID NO: 13607 - protein, 9 aa, synthetic construct
GGDGADQFL

SEQ ID NO: 13608 - protein, 9 aa, synthetic construct
GGEGADALS

SEQ ID NO: 13609 - protein, 9 aa, synthetic construct
GGGGSDVLT

SEQ ID NO: 13610 - protein, 9 aa, synthetic construct
GGDGADYLL

SEQ ID NO: 13611 - protein, 9 aa, synthetic construct
GGAGDDEIE

SEQ ID NO: 13612 - protein, 9 aa, synthetic construct
GGGGDDFVN

SEQ ID NO: 13613 - protein, 9 aa, synthetic construct
GGVGIDTLY

SEQ ID NO: 13614 - protein, 9 aa, synthetic construct
GGDGADTVT

SEQ ID NO: 13615 - protein, 9 aa, synthetic construct
GGHGKDTLK

SEQ ID NO: 13616 - protein, 9 aa, synthetic construct
GGMGDDALH

SEQ ID NO: 13617 - protein, 9 aa, synthetic construct
GGYGNDKLT

SEQ ID NO: 13618 - protein, 9 aa, synthetic construct
GGVGNDTIT

SEQ ID NO: 13619 - protein, 9 aa, synthetic construct
GGNGRDRLF

SEQ ID NO: 13620 - protein, 9 aa, synthetic construct
GGAGDDHLA

SEQ ID NO: 13621 - protein, 9 aa, synthetic construct
GGGGSDTYK

SEQ ID NO: 13622 - protein, 9 aa, synthetic construct
GGVGLDLLS

SEQ ID NO: 13623 - protein, 9 aa, synthetic construct
GGAGTDSLG

SEQ ID NO: 13624 - protein, 9 aa, synthetic construct
GGVGIDSMA

SEQ ID NO: 13625 - protein, 9 aa, synthetic construct
GGNGRDRAF

SEQ ID NO: 13626 - protein, 9 aa, synthetic construct
GGDGTDTIH

SEQ ID NO: 13627 - protein, 9 aa, synthetic construct
GGDGADRIA

SEQ ID NO: 13628 - protein, 9 aa, synthetic construct
GGVGLDQLF

SEQ ID NO: 13629 - protein, 9 aa, synthetic construct
GGDGADTMF

SEQ ID NO: 13630 - protein, 9 aa, synthetic construct
GGVGNDSIS

SEQ ID NO: 13631 - protein, 9 aa, synthetic construct
GGNGRDRIF

SEQ ID NO: 13632 - protein, 9 aa, synthetic construct
GGSGTDFLY

SEQ ID NO: 13633 - protein, 9 aa, synthetic construct
GGGGSDRLI

SEQ ID NO: 13634 - protein, 9 aa, synthetic construct
GGLGHDTLS

SEQ ID NO: 13635 - protein, 9 aa, synthetic construct
GGVGNDVFI

SEQ ID NO: 13636 - protein, 9 aa, synthetic construct
GGKGDDILA

SEQ ID NO: 13637 - protein, 9 aa, synthetic construct
GGQGADILL

SEQ ID NO: 13638 - protein, 9 aa, synthetic construct
GGGGSDVVI

SEQ ID NO: 13639 - protein, 9 aa, synthetic construct
GGYGNDLLS

SEQ ID NO: 13640 - protein, 9 aa, synthetic construct
GGLGGDYLY

SEQ ID NO: 13641 - protein, 9 aa, synthetic construct
GGAGDDDLH

SEQ ID NO: 13642 - protein, 9 aa, synthetic construct
GGNGRDQLF

SEQ ID NO: 13643 - protein, 9 aa, synthetic construct
GGLGEDTLN

SEQ ID NO: 13644 - protein, 9 aa, synthetic construct
GGNGNDELS

SEQ ID NO: 13645 - protein, 9 aa, synthetic construct
GGAGKDVLE

SEQ ID NO: 13646 - protein, 9 aa, synthetic construct
GGEGSDLIR

SEQ ID NO: 13647 - protein, 9 aa, synthetic construct
GGAGTDLVS

SEQ ID NO: 13648 - protein, 9 aa, synthetic construct
GGNGNDELT

SEQ ID NO: 13649 - protein, 9 aa, synthetic construct
GGAGTDSLN

SEQ ID NO: 13650 - protein, 9 aa, synthetic construct
GGLGHDAVI

SEQ ID NO: 13651 - protein, 9 aa, synthetic construct
GGDGGDTMG

SEQ ID NO: 13652 - protein, 9 aa, synthetic construct
GGKGDDKLQ

SEQ ID NO: 13653 - protein, 9 aa, synthetic construct
GGDGKDILS

SEQ ID NO: 13654 - protein, 9 aa, synthetic construct
GGSGRDQME

SEQ ID NO: 13655 - protein, 9 aa, synthetic construct
GGGGSDVMN

SEQ ID NO: 13656 - protein, 9 aa, synthetic construct
GGSGQDYMD

SEQ ID NO: 13657 - protein, 9 aa, synthetic construct
GGEGQDSLS

SEQ ID NO: 13658 - protein, 9 aa, synthetic construct
GGKGDDQMY

SEQ ID NO: 13659 - protein, 9 aa, synthetic construct
GGSGTDTIS

SEQ ID NO: 13660 - protein, 9 aa, synthetic construct
GGDGTDTAD

SEQ ID NO: 13661 - protein, 9 aa, synthetic construct
GGKGEDDLR

SEQ ID NO: 13662 - protein, 9 aa, synthetic construct
GGVGNDSLE

SEQ ID NO: 13663 - protein, 9 aa, synthetic construct
GGSGTDFLD

SEQ ID NO: 13664 - protein, 9 aa, synthetic construct
GGEGADALN

SEQ ID NO: 13665 - protein, 9 aa, synthetic construct
GGDGADRFS

SEQ ID NO: 13666 - protein, 9 aa, synthetic construct
GGKGFDTLD

SEQ ID NO: 13667 - protein, 9 aa, synthetic construct
GGLGQDTLS

SEQ ID NO: 13668 - protein, 9 aa, synthetic construct
GGQGDDTIG

SEQ ID NO: 13669 - protein, 9 aa, synthetic construct
GGAGDDIFL

SEQ ID NO: 13670 - protein, 9 aa, synthetic construct
GGAGDDHLN

SEQ ID NO: 13671 - protein, 9 aa, synthetic construct
GGAGSDVLM

SEQ ID NO: 13672 - protein, 9 aa, synthetic construct
GGMGNDTLF

SEQ ID NO: 13673 - protein, 9 aa, synthetic construct
GGDGADNLV

SEQ ID NO: 13674 - protein, 9 aa, synthetic construct
GGNGNDSVS

SEQ ID NO: 13675 - protein, 9 aa, synthetic construct
GGQGADILI

SEQ ID NO: 13676 - protein, 9 aa, synthetic construct
GGNGRDRIN

SEQ ID NO: 13677 - protein, 9 aa, synthetic construct
GGKGADLLS

SEQ ID NO: 13678 - protein, 9 aa, synthetic construct
GGGGSDRLE

SEQ ID NO: 13679 - protein, 9 aa, synthetic construct
GGVGIDSMS

SEQ ID NO: 13680 - protein, 9 aa, synthetic construct
GGQGDDVLN

SEQ ID NO: 13681 - protein, 9 aa, synthetic construct
GGGGEDILQ

SEQ ID NO: 13682 - protein, 9 aa, synthetic construct
GGDGIDWVD

SEQ ID NO: 13683 - protein, 9 aa, synthetic construct
GGEGDDFLW

SEQ ID NO: 13684 - protein, 9 aa, synthetic construct
GGAGTDSLA

SEQ ID NO: 13685 - protein, 9 aa, synthetic construct
GGAGTDMAS

SEQ ID NO: 13686 - protein, 9 aa, synthetic construct
GGGGHDVLQ

SEQ ID NO: 13687 - protein, 9 aa, synthetic construct
GGLGNDTIW

SEQ ID NO: 13688 - protein, 9 aa, synthetic construct
GGEGFDIAD

SEQ ID NO: 13689 - protein, 9 aa, synthetic construct
GGFGNDLLR

SEQ ID NO: 13690 - protein, 9 aa, synthetic construct
GGGGSDLLY

SEQ ID NO: 13691 - protein, 9 aa, synthetic construct
GGQGDDVIV

SEQ ID NO: 13692 - protein, 9 aa, synthetic construct
GGFGEDSIM

SEQ ID NO: 13693 - protein, 9 aa, synthetic construct
GGGGRDSLF

SEQ ID NO: 13694 - protein, 9 aa, synthetic construct
GGVGNDTFI

SEQ ID NO: 13695 - protein, 9 aa, synthetic construct
GGAGLDFAD

SEQ ID NO: 13696 - protein, 9 aa, synthetic construct
GGDGDDWMD

SEQ ID NO: 13697 - protein, 9 aa, synthetic construct
GGNGRDTLE

SEQ ID NO: 13698 - protein, 9 aa, synthetic construct
GGDGADQLQ

SEQ ID NO: 13699 - protein, 9 aa, synthetic construct
GGDGADQLN

SEQ ID NO: 13700 - protein, 9 aa, synthetic construct
GGSGRDLLM

SEQ ID NO: 13701 - protein, 9 aa, synthetic construct
GGGGHDIAS

SEQ ID NO: 13702 - protein, 9 aa, synthetic construct
GGNGLDTLK

SEQ ID NO: 13703 - protein, 9 aa, synthetic construct
GGDGADQIS

SEQ ID NO: 13704 - protein, 9 aa, synthetic construct
GGLGEDTFV

SEQ ID NO: 13705 - protein, 9 aa, synthetic construct
GGKGADRLE

SEQ ID NO: 13706 - protein, 9 aa, synthetic construct
GGLGEDTIF

SEQ ID NO: 13707 - protein, 9 aa, synthetic construct
GGEGDDVIR

SEQ ID NO: 13708 - protein, 9 aa, synthetic construct
GGEGKDTLA

SEQ ID NO: 13709 - protein, 9 aa, synthetic construct
GGAGTDRLQ

SEQ ID NO: 13710 - protein, 9 aa, synthetic construct
GGDGDDWLT

SEQ ID NO: 13711 - protein, 9 aa, synthetic construct
GGYGVDEII

SEQ ID NO: 13712 - protein, 9 aa, synthetic construct
GGDGADYLH

SEQ ID NO: 13713 - protein, 9 aa, synthetic construct
GGLGNDTMD

SEQ ID NO: 13714 - protein, 9 aa, synthetic construct
GGQGADAID

SEQ ID NO: 13715 - protein, 9 aa, synthetic construct
GGSGTDTLK

SEQ ID NO: 13716 - protein, 9 aa, synthetic construct
GGEGFDLLT

SEQ ID NO: 13717 - protein, 9 aa, synthetic construct
GGQGDDTYL

SEQ ID NO: 13718 - protein, 9 aa, synthetic construct
GGLGVDSLY

SEQ ID NO: 13719 - protein, 9 aa, synthetic construct
GGSGRDLLK

SEQ ID NO: 13720 - protein, 9 aa, synthetic construct
GGVGNDTVG

SEQ ID NO: 13721 - protein, 9 aa, synthetic construct
GGEGLDTFT

SEQ ID NO: 13722 - protein, 9 aa, synthetic construct
GGLGHDSID

SEQ ID NO: 13723 - protein, 9 aa, synthetic construct
GGNGRDVLL

SEQ ID NO: 13724 - protein, 9 aa, synthetic construct
GGAGADHLA

SEQ ID NO: 13725 - protein, 9 aa, synthetic construct
GGLGEDTFL

SEQ ID NO: 13726 - protein, 9 aa, synthetic construct
GGQGDDTMT

SEQ ID NO: 13727 - protein, 9 aa, synthetic construct
GGQGDDTMV

SEQ ID NO: 13728 - protein, 9 aa, synthetic construct
GGEGDDFVL

SEQ ID NO: 13729 - protein, 9 aa, synthetic construct
GGVGNDTIF

SEQ ID NO: 13730 - protein, 9 aa, synthetic construct
GGLGHDNMT

SEQ ID NO: 13731 - protein, 9 aa, synthetic construct
GGAGTDRLV

SEQ ID NO: 13732 - protein, 9 aa, synthetic construct
GGAGDDDMN

SEQ ID NO: 13733 - protein, 9 aa, synthetic construct
GGGGSDVIY

SEQ ID NO: 13734 - protein, 9 aa, synthetic construct
GGEGNDTVR

SEQ ID NO: 13735 - protein, 9 aa, synthetic construct
GGGGEDDYF

SEQ ID NO: 13736 - protein, 9 aa, synthetic construct
GGLGHDRLD

SEQ ID NO: 13737 - protein, 9 aa, synthetic construct
GGNGNDFLQ

SEQ ID NO: 13738 - protein, 9 aa, synthetic construct
GGYGVDLLN

SEQ ID NO: 13739 - protein, 9 aa, synthetic construct
GGLGVDTAF

SEQ ID NO: 13740 - protein, 9 aa, synthetic construct
GGGGRDSLQ

SEQ ID NO: 13741 - protein, 9 aa, synthetic construct
GGVGNDTMD

SEQ ID NO: 13742 - protein, 9 aa, synthetic construct
GGSGNDNIQ

SEQ ID NO: 13743 - protein, 9 aa, synthetic construct
GGAGTDRLA

SEQ ID NO: 13744 - protein, 9 aa, synthetic construct
GGKGDDIYY

SEQ ID NO: 13745 - protein, 9 aa, synthetic construct
GGAGADALE

SEQ ID NO: 13746 - protein, 9 aa, synthetic construct
GGVGKDLLR

SEQ ID NO: 13747 - protein, 9 aa, synthetic construct
GGAGTDRIF

SEQ ID NO: 13748 - protein, 9 aa, synthetic construct
GGAGTDRIV

SEQ ID NO: 13749 - protein, 9 aa, synthetic construct
GGHGDDRLY

SEQ ID NO: 13750 - protein, 9 aa, synthetic construct
GGLGNDYLH

SEQ ID NO: 13751 - protein, 9 aa, synthetic construct
GGAGLDELR

SEQ ID NO: 13752 - protein, 9 aa, synthetic construct
GGNGRDVIY

SEQ ID NO: 13753 - protein, 9 aa, synthetic construct
GGAGTDRAQ

SEQ ID NO: 13754 - protein, 9 aa, synthetic construct
GGYGVDHIH

SEQ ID NO: 13755 - protein, 9 aa, synthetic construct
GGDGNDWFD

SEQ ID NO: 13756 - protein, 9 aa, synthetic construct
GGEGRDHLT

SEQ ID NO: 13757 - protein, 9 aa, synthetic construct
GGEGRDHLY

SEQ ID NO: 13758 - protein, 9 aa, synthetic construct
GGDGADQIT

SEQ ID NO: 13759 - protein, 9 aa, synthetic construct
GGAGADHID

SEQ ID NO: 13760 - protein, 9 aa, synthetic construct
GGHGDDSLE

SEQ ID NO: 13761 - protein, 9 aa, synthetic construct
GGLGHDQLV

SEQ ID NO: 13762 - protein, 9 aa, synthetic construct
GGVGNDTIL

SEQ ID NO: 13763 - protein, 9 aa, synthetic construct
GGFGNDALF

SEQ ID NO: 13764 - protein, 9 aa, synthetic construct
GGKGDDQLF

SEQ ID NO: 13765 - protein, 9 aa, synthetic construct
GGLGQDTLF

SEQ ID NO: 13766 - protein, 9 aa, synthetic construct
GGGGEDVLR

SEQ ID NO: 13767 - protein, 9 aa, synthetic construct
GGQGDDTVT

SEQ ID NO: 13768 - protein, 9 aa, synthetic construct
GGEGNDTVN

SEQ ID NO: 13769 - protein, 9 aa, synthetic construct
GGVGNDTVI

SEQ ID NO: 13770 - protein, 9 aa, synthetic construct
GGAGDDEAF

SEQ ID NO: 13771 - protein, 9 aa, synthetic construct
GGNGDDMLR

SEQ ID NO: 13772 - protein, 9 aa, synthetic construct
GGKGDDQLY

SEQ ID NO: 13773 - protein, 9 aa, synthetic construct
GGAGDDIAY

SEQ ID NO: 13774 - protein, 9 aa, synthetic construct
GGNGNDGFD

SEQ ID NO: 13775 - protein, 9 aa, synthetic construct
GGNGNDFID

SEQ ID NO: 13776 - protein, 9 aa, synthetic construct
GGQGDDTLH

SEQ ID NO: 13777 - protein, 9 aa, synthetic construct
GGEGRDIFL

SEQ ID NO: 13778 - protein, 9 aa, synthetic construct
GGEGNDTVV

SEQ ID NO: 13779 - protein, 9 aa, synthetic construct
GGNGRDSLN

SEQ ID NO: 13780 - protein, 9 aa, synthetic construct
GGLGHDILD

SEQ ID NO: 13781 - protein, 9 aa, synthetic construct
GGSGTDTVS

SEQ ID NO: 13782 - protein, 9 aa, synthetic construct
GGQGDDTLM

SEQ ID NO: 13783 - protein, 9 aa, synthetic construct
GGLGHDILN

SEQ ID NO: 13784 - protein, 9 aa, synthetic construct
GGPGTDTAV

SEQ ID NO: 13785 - protein, 9 aa, synthetic construct
GGDGKDGLR

SEQ ID NO: 13786 - protein, 9 aa, synthetic construct
GGQGADDLT

SEQ ID NO: 13787 - protein, 9 aa, synthetic construct
GGNGNDTAT

SEQ ID NO: 13788 - protein, 9 aa, synthetic construct
GGSGRDTMI

SEQ ID NO: 13789 - protein, 9 aa, synthetic construct
GGDGNDVVQ

SEQ ID NO: 13790 - protein, 9 aa, synthetic construct
GGDGNDTVV

SEQ ID NO: 13791 - protein, 9 aa, synthetic construct
GGDGDDVVF

SEQ ID NO: 13792 - protein, 9 aa, synthetic construct
GGLGHDHLE

SEQ ID NO: 13793 - protein, 9 aa, synthetic construct
GGLGNDYYI

SEQ ID NO: 13794 - protein, 9 aa, synthetic construct
GGHGDDRLF

SEQ ID NO: 13795 - protein, 9 aa, synthetic construct
GGGGSDVLR

SEQ ID NO: 13796 - protein, 9 aa, synthetic construct
GGDGADTMD

SEQ ID NO: 13797 - protein, 9 aa, synthetic construct
GGAGTDSAD

SEQ ID NO: 13798 - protein, 9 aa, synthetic construct
GGDGKDIFV

SEQ ID NO: 13799 - protein, 9 aa, synthetic construct
GGVGKDTLD

SEQ ID NO: 13800 - protein, 9 aa, synthetic construct
GGDGGDALQ

SEQ ID NO: 13801 - protein, 9 aa, synthetic construct
GGGGSDNFV

SEQ ID NO: 13802 - protein, 9 aa, synthetic construct
GGLGHDHLQ

SEQ ID NO: 13803 - protein, 9 aa, synthetic construct
GGAGMDILN

SEQ ID NO: 13804 - protein, 9 aa, synthetic construct
GGAGKDIFQ

SEQ ID NO: 13805 - protein, 9 aa, synthetic construct
GGDGADTLW

SEQ ID NO: 13806 - protein, 9 aa, synthetic construct
GGPGTDSLV

SEQ ID NO: 13807 - protein, 9 aa, synthetic construct
GGNGNDGID

SEQ ID NO: 13808 - protein, 9 aa, synthetic construct
GGKGFDSYV

SEQ ID NO: 13809 - protein, 9 aa, synthetic construct
GGLGNDTMQ

SEQ ID NO: 13810 - protein, 9 aa, synthetic construct
GGAGKDTLH

SEQ ID NO: 13811 - protein, 9 aa, synthetic construct
GGQGADALF

SEQ ID NO: 13812 - protein, 9 aa, synthetic construct
GGLGNDTMF

SEQ ID NO: 13813 - protein, 9 aa, synthetic construct
GGAGADALM

SEQ ID NO: 13814 - protein, 9 aa, synthetic construct
GGDGTDTAL

SEQ ID NO: 13815 - protein, 9 aa, synthetic construct
GGDGNDTVW

SEQ ID NO: 13816 - protein, 9 aa, synthetic construct
GGSGNDSFF

SEQ ID NO: 13817 - protein, 9 aa, synthetic construct
GGGGRDQLF

SEQ ID NO: 13818 - protein, 9 aa, synthetic construct
GGEGDDRLK

SEQ ID NO: 13819 - protein, 9 aa, synthetic construct
GGYGNDILY

SEQ ID NO: 13820 - protein, 9 aa, synthetic construct
GGLGHDSLN

SEQ ID NO: 13821 - protein, 9 aa, synthetic construct
GGGGEDVLV

SEQ ID NO: 13822 - protein, 9 aa, synthetic construct
GGKGDDKLF

SEQ ID NO: 13823 - protein, 9 aa, synthetic construct
GGEGDDFYS

SEQ ID NO: 13824 - protein, 9 aa, synthetic construct
GGEGMDIAD

SEQ ID NO: 13825 - protein, 9 aa, synthetic construct
GGDGADQLT

SEQ ID NO: 13826 - protein, 9 aa, synthetic construct
GGYGNDEIY

SEQ ID NO: 13827 - protein, 9 aa, synthetic construct
GGGGSDQLH

SEQ ID NO: 13828 - protein, 9 aa, synthetic construct
GGNGNDFVW

SEQ ID NO: 13829 - protein, 9 aa, synthetic construct
GGSGRDLLR

SEQ ID NO: 13830 - protein, 9 aa, synthetic construct
GGLGQDTLI

SEQ ID NO: 13831 - protein, 9 aa, synthetic construct
GGSGRDQLF

SEQ ID NO: 13832 - protein, 9 aa, synthetic construct
GGAGKDILF

SEQ ID NO: 13833 - protein, 9 aa, synthetic construct
GGSGTDALV

SEQ ID NO: 13834 - protein, 9 aa, synthetic construct
GGDGIDYLT

SEQ ID NO: 13835 - protein, 9 aa, synthetic construct
GGQGDDTLQ

SEQ ID NO: 13836 - protein, 9 aa, synthetic construct
GGVGNDTYF

SEQ ID NO: 13837 - protein, 9 aa, synthetic construct
GGSGTDTLE

SEQ ID NO: 13838 - protein, 9 aa, synthetic construct
GGGGEDALW

SEQ ID NO: 13839 - protein, 9 aa, synthetic construct
GGDGADQMN

SEQ ID NO: 13840 - protein, 9 aa, synthetic construct
GGSGNDNID

SEQ ID NO: 13841 - protein, 9 aa, synthetic construct
GGVGNDSVN

SEQ ID NO: 13842 - protein, 9 aa, synthetic construct
GGGGLDTVD

SEQ ID NO: 13843 - protein, 9 aa, synthetic construct
GGDGADTVE

SEQ ID NO: 13844 - protein, 9 aa, synthetic construct
GGDGKDVVS

SEQ ID NO: 13845 - protein, 9 aa, synthetic construct
GGSGRDTMA

SEQ ID NO: 13846 - protein, 9 aa, synthetic construct
GGAGADGLS

SEQ ID NO: 13847 - protein, 9 aa, synthetic construct
GGDGTDTAI

SEQ ID NO: 13848 - protein, 9 aa, synthetic construct
GGEGADGLY

SEQ ID NO: 13849 - protein, 9 aa, synthetic construct
GGDGDDVYY

SEQ ID NO: 13850 - protein, 9 aa, synthetic construct
GGGGNDAMH

SEQ ID NO: 13851 - protein, 9 aa, synthetic construct
GGAGKDVFQ

SEQ ID NO: 13852 - protein, 9 aa, synthetic construct
GGAGDDFIM

SEQ ID NO: 13853 - protein, 9 aa, synthetic construct
GGVGNDKLY

SEQ ID NO: 13854 - protein, 9 aa, synthetic construct
GGSGRDRLI

SEQ ID NO: 13855 - protein, 9 aa, synthetic construct
GGAGKDEFV

SEQ ID NO: 13856 - protein, 9 aa, synthetic construct
GGYGNDTYI

SEQ ID NO: 13857 - protein, 9 aa, synthetic construct
GGAGADHMT

SEQ ID NO: 13858 - protein, 9 aa, synthetic construct
GGDGADSLM

SEQ ID NO: 13859 - protein, 9 aa, synthetic construct
GGGGHDHLY

SEQ ID NO: 13860 - protein, 9 aa, synthetic construct
GGAGADEMY

SEQ ID NO: 13861 - protein, 9 aa, synthetic construct
GGVGNDKVF

SEQ ID NO: 13862 - protein, 9 aa, synthetic construct
GGEGQDLLV

SEQ ID NO: 13863 - protein, 9 aa, synthetic construct
GGVGNDLFY

SEQ ID NO: 13864 - protein, 9 aa, synthetic construct
GGAGDDFIR

SEQ ID NO: 13865 - protein, 9 aa, synthetic construct
GGGGDDEIH

SEQ ID NO: 13866 - protein, 9 aa, synthetic construct
GGAGKDDVD

SEQ ID NO: 13867 - protein, 9 aa, synthetic construct
GGAGSDYFV

SEQ ID NO: 13868 - protein, 9 aa, synthetic construct
GGYGNDTLV

SEQ ID NO: 13869 - protein, 9 aa, synthetic construct
GGDGKDTIF

SEQ ID NO: 13870 - protein, 9 aa, synthetic construct
GGYGNDTLH

SEQ ID NO: 13871 - protein, 9 aa, synthetic construct
GGGGSDTIN

SEQ ID NO: 13872 - protein, 9 aa, synthetic construct
GGAGDDFIF

SEQ ID NO: 13873 - protein, 9 aa, synthetic construct
GGDGDDMLA

SEQ ID NO: 13874 - protein, 9 aa, synthetic construct
GGDGKDNLS

SEQ ID NO: 13875 - protein, 9 aa, synthetic construct
GGVGNDKLV

SEQ ID NO: 13876 - protein, 9 aa, synthetic construct
GGDGTDTVT

SEQ ID NO: 13877 - protein, 9 aa, synthetic construct
GGGGDDELN

SEQ ID NO: 13878 - protein, 9 aa, synthetic construct
GGNGNDVYV

SEQ ID NO: 13879 - protein, 9 aa, synthetic construct
GGQGDDEID

SEQ ID NO: 13880 - protein, 9 aa, synthetic construct
GGDGADSMS

SEQ ID NO: 13881 - protein, 9 aa, synthetic construct
GGDGADSMN

SEQ ID NO: 13882 - protein, 9 aa, synthetic construct
GGDGADSMF

SEQ ID NO: 13883 - protein, 9 aa, synthetic construct
GGSGRDFFL

SEQ ID NO: 13884 - protein, 9 aa, synthetic construct
GGDGADTIA

SEQ ID NO: 13885 - protein, 9 aa, synthetic construct
GGEGADELH

SEQ ID NO: 13886 - protein, 9 aa, synthetic construct
GGQGDDDLS

SEQ ID NO: 13887 - protein, 9 aa, synthetic construct
GGSGTDRLY

SEQ ID NO: 13888 - protein, 9 aa, synthetic construct
GGNGNDVYY

SEQ ID NO: 13889 - protein, 9 aa, synthetic construct
GGHGHDKMY

SEQ ID NO: 13890 - protein, 9 aa, synthetic construct
GGVGNDKLH

SEQ ID NO: 13891 - protein, 9 aa, synthetic construct
GGYGNDVLH

SEQ ID NO: 13892 - protein, 9 aa, synthetic construct
GGGGSDTFS

SEQ ID NO: 13893 - protein, 9 aa, synthetic construct
GGYGNDVLD

SEQ ID NO: 13894 - protein, 9 aa, synthetic construct
GGAGDDFYL

SEQ ID NO: 13895 - protein, 9 aa, synthetic construct
GGQGDDDLD

SEQ ID NO: 13896 - protein, 9 aa, synthetic construct
GGSGNDRAF

SEQ ID NO: 13897 - protein, 9 aa, synthetic construct
GGVGNDKLD

SEQ ID NO: 13898 - protein, 9 aa, synthetic construct
GGGGSDSLT

SEQ ID NO: 13899 - protein, 9 aa, synthetic construct
GGYGNDTYY

SEQ ID NO: 13900 - protein, 9 aa, synthetic construct
GGEGQDKVT

SEQ ID NO: 13901 - protein, 9 aa, synthetic construct
GGAGADEFE

SEQ ID NO: 13902 - protein, 9 aa, synthetic construct
GGAGKDTYN

SEQ ID NO: 13903 - protein, 9 aa, synthetic construct
GGEGDDFIL

SEQ ID NO: 13904 - protein, 9 aa, synthetic construct
GGAGTDIAS

SEQ ID NO: 13905 - protein, 9 aa, synthetic construct
GGAGKDDLW

SEQ ID NO: 13906 - protein, 9 aa, synthetic construct
GGNGNDDIW

SEQ ID NO: 13907 - protein, 9 aa, synthetic construct
GGYGNDTIE

SEQ ID NO: 13908 - protein, 9 aa, synthetic construct
GGDGTDTVD

SEQ ID NO: 13909 - protein, 9 aa, synthetic construct
GGNGNDDLF

SEQ ID NO: 13910 - protein, 9 aa, synthetic construct
GGSGNDRIA

SEQ ID NO: 13911 - protein, 9 aa, synthetic construct
GGAGSDYAI

SEQ ID NO: 13912 - protein, 9 aa, synthetic construct
GGVGNDLLT

SEQ ID NO: 13913 - protein, 9 aa, synthetic construct
GGLGNDVIS

SEQ ID NO: 13914 - protein, 9 aa, synthetic construct
GGVGNDLLV

SEQ ID NO: 13915 - protein, 9 aa, synthetic construct
GGAGDDGIR

SEQ ID NO: 13916 - protein, 9 aa, synthetic construct
GGEGDDVYV

SEQ ID NO: 13917 - protein, 9 aa, synthetic construct
GGDGKDTLE

SEQ ID NO: 13918 - protein, 9 aa, synthetic construct
GGQGDDLYI

SEQ ID NO: 13919 - protein, 9 aa, synthetic construct
GGNGQDTID

SEQ ID NO: 13920 - protein, 9 aa, synthetic construct
GGDGNDVMY

SEQ ID NO: 13921 - protein, 9 aa, synthetic construct
GGVGNDALY

SEQ ID NO: 13922 - protein, 9 aa, synthetic construct
GGNGQDTIT

SEQ ID NO: 13923 - protein, 9 aa, synthetic construct
GGDGDDMIR

SEQ ID NO: 13924 - protein, 9 aa, synthetic construct
GGFGLDFLD

SEQ ID NO: 13925 - protein, 9 aa, synthetic construct
GGNGMDSLA

SEQ ID NO: 13926 - protein, 9 aa, synthetic construct
GGLGGDSLT

SEQ ID NO: 13927 - protein, 9 aa, synthetic construct
GGLGGDRLV

SEQ ID NO: 13928 - protein, 9 aa, synthetic construct
GGDGADSII

SEQ ID NO: 13929 - protein, 9 aa, synthetic construct
GGGGRDRLR

SEQ ID NO: 13930 - protein, 9 aa, synthetic construct
GGKGDDILQ

SEQ ID NO: 13931 - protein, 9 aa, synthetic construct
GGYGNDTIS

SEQ ID NO: 13932 - protein, 9 aa, synthetic construct
GGNGQDQLF

SEQ ID NO: 13933 - protein, 9 aa, synthetic construct
GGDGTDTVR

SEQ ID NO: 13934 - protein, 9 aa, synthetic construct
GGDGHDGLR

SEQ ID NO: 13935 - protein, 9 aa, synthetic construct
GGEGADELQ

SEQ ID NO: 13936 - protein, 9 aa, synthetic construct
GGDGDDWIN

SEQ ID NO: 13937 - protein, 9 aa, synthetic construct
GGLGGDQLN

SEQ ID NO: 13938 - protein, 9 aa, synthetic construct
GGDGDDVVT

SEQ ID NO: 13939 - protein, 9 aa, synthetic construct
GGLGQDVLI

SEQ ID NO: 13940 - protein, 9 aa, synthetic construct
GGAGADDVD

SEQ ID NO: 13941 - protein, 9 aa, synthetic construct
GGNGNDVMR

SEQ ID NO: 13942 - protein, 9 aa, synthetic construct
GGVGNDLIY

SEQ ID NO: 13943 - protein, 9 aa, synthetic construct
GGLGGDRLD

SEQ ID NO: 13944 - protein, 9 aa, synthetic construct
GGNGNDVML

SEQ ID NO: 13945 - protein, 9 aa, synthetic construct
GGAGADDMT

SEQ ID NO: 13946 - protein, 9 aa, synthetic construct
GGQGADVLT

SEQ ID NO: 13947 - protein, 9 aa, synthetic construct
GGDGTDYLM

SEQ ID NO: 13948 - protein, 9 aa, synthetic construct
GGEGFDWAS

SEQ ID NO: 13949 - protein, 9 aa, synthetic construct
GGSGTDSIL

SEQ ID NO: 13950 - protein, 9 aa, synthetic construct
GGQGADVLL

SEQ ID NO: 13951 - protein, 9 aa, synthetic construct
GGLGNDWLH

SEQ ID NO: 13952 - protein, 9 aa, synthetic construct
GGDGADSMT

SEQ ID NO: 13953 - protein, 9 aa, synthetic construct
GGFGNDNID

SEQ ID NO: 13954 - protein, 9 aa, synthetic construct
GGHGEDLLN

SEQ ID NO: 13955 - protein, 9 aa, synthetic construct
GGDGFDVAS

SEQ ID NO: 13956 - protein, 9 aa, synthetic construct
GGSGRDRLW

SEQ ID NO: 13957 - protein, 9 aa, synthetic construct
GGAGTDALH

SEQ ID NO: 13958 - protein, 9 aa, synthetic construct
GGAGADELA

SEQ ID NO: 13959 - protein, 9 aa, synthetic construct
GGGGKDDLL

SEQ ID NO: 13960 - protein, 9 aa, synthetic construct
GGLGNDVYL

SEQ ID NO: 13961 - protein, 9 aa, synthetic construct
GGGGEDRLS

SEQ ID NO: 13962 - protein, 9 aa, synthetic construct
GGKGDDLLK

SEQ ID NO: 13963 - protein, 9 aa, synthetic construct
GGYGNDWIS

SEQ ID NO: 13964 - protein, 9 aa, synthetic construct
GGAGKDWVT

SEQ ID NO: 13965 - protein, 9 aa, synthetic construct
GGEGDDVIV

SEQ ID NO: 13966 - protein, 9 aa, synthetic construct
GGAGSDYLY

SEQ ID NO: 13967 - protein, 9 aa, synthetic construct
GGGGDDDIR

SEQ ID NO: 13968 - protein, 9 aa, synthetic construct
GGDGADTFK

SEQ ID NO: 13969 - protein, 9 aa, synthetic construct
GGAGADEIW

SEQ ID NO: 13970 - protein, 9 aa, synthetic construct
GGAGADEIT

SEQ ID NO: 13971 - protein, 9 aa, synthetic construct
GGDGDDAIG

SEQ ID NO: 13972 - protein, 9 aa, synthetic construct
GGAGTDALY

SEQ ID NO: 13973 - protein, 9 aa, synthetic construct
GGAGDDFLQ

SEQ ID NO: 13974 - protein, 9 aa, synthetic construct
GGAGKDYLD

SEQ ID NO: 13975 - protein, 9 aa, synthetic construct
GGDGTDVYD

SEQ ID NO: 13976 - protein, 9 aa, synthetic construct
GGDGADTFN

SEQ ID NO: 13977 - protein, 9 aa, synthetic construct
GGVGNDIIY

SEQ ID NO: 13978 - protein, 9 aa, synthetic construct
GGHGEDTLN

SEQ ID NO: 13979 - protein, 9 aa, synthetic construct
GGEGADMLD

SEQ ID NO: 13980 - protein, 9 aa, synthetic construct
GGVGNDFLF

SEQ ID NO: 13981 - protein, 9 aa, synthetic construct
GGAGADELE

SEQ ID NO: 13982 - protein, 9 aa, synthetic construct
GGNGNDYIN

SEQ ID NO: 13983 - protein, 9 aa, synthetic construct
GGSGNDQMF

SEQ ID NO: 13984 - protein, 9 aa, synthetic construct
GGLGNDVVV

SEQ ID NO: 13985 - protein, 9 aa, synthetic construct
GGKGEDTLY

SEQ ID NO: 13986 - protein, 9 aa, synthetic construct
GGQGDDILS

SEQ ID NO: 13987 - protein, 9 aa, synthetic construct
GGGGSDTAS

SEQ ID NO: 13988 - protein, 9 aa, synthetic construct
GGLGNDVVE

SEQ ID NO: 13989 - protein, 9 aa, synthetic construct
GGDGTDVLS

SEQ ID NO: 13990 - protein, 9 aa, synthetic construct
GGQGDDILT

SEQ ID NO: 13991 - protein, 9 aa, synthetic construct
GGSGTDRLA

SEQ ID NO: 13992 - protein, 9 aa, synthetic construct
GGQGDDILE

SEQ ID NO: 13993 - protein, 9 aa, synthetic construct
GGKGADMMR

SEQ ID NO: 13994 - protein, 9 aa, synthetic construct
GGNGNDAFD

SEQ ID NO: 13995 - protein, 9 aa, synthetic construct
GGQGDDIIV

SEQ ID NO: 13996 - protein, 9 aa, synthetic construct
GGLGFDVLT

SEQ ID NO: 13997 - protein, 9 aa, synthetic construct
GGQGDDIII

SEQ ID NO: 13998 - protein, 9 aa, synthetic construct
GGQGDDIIF

SEQ ID NO: 13999 - protein, 9 aa, synthetic construct
GGHGEDVLN

SEQ ID NO: 14000 - protein, 9 aa, synthetic construct
GGEGLDWLL

SEQ ID NO: 14001 - protein, 9 aa, synthetic construct
GGGGDDAVD

SEQ ID NO: 14002 - protein, 9 aa, synthetic construct
GGVGNDHLD

SEQ ID NO: 14003 - protein, 9 aa, synthetic construct
GGAGADEME

SEQ ID NO: 14004 - protein, 9 aa, synthetic construct
GGGGDDALR

SEQ ID NO: 14005 - protein, 9 aa, synthetic construct
GGAGSDYIN

SEQ ID NO: 14006 - protein, 9 aa, synthetic construct
GGAGADEID

SEQ ID NO: 14007 - protein, 9 aa, synthetic construct
GGGGSDLIR

SEQ ID NO: 14008 - protein, 9 aa, synthetic construct
GGGGDDDLF

SEQ ID NO: 14009 - protein, 9 aa, synthetic construct
GGAGSDYLE

SEQ ID NO: 14010 - protein, 9 aa, synthetic construct
GGQGDDFIG

SEQ ID NO: 14011 - protein, 9 aa, synthetic construct
GGLGGDEYL

SEQ ID NO: 14012 - protein, 9 aa, synthetic construct
GGGGSDSMD

SEQ ID NO: 14013 - protein, 9 aa, synthetic construct
GGYGNDVLS

SEQ ID NO: 14014 - protein, 9 aa, synthetic construct
GGVGNDELD

SEQ ID NO: 14015 - protein, 9 aa, synthetic construct
GGAGKDWLK

SEQ ID NO: 14016 - protein, 9 aa, synthetic construct
GGDGKDRLE

SEQ ID NO: 14017 - protein, 9 aa, synthetic construct
GGDGADTFY

SEQ ID NO: 14018 - protein, 9 aa, synthetic construct
GGGGDDDIT

SEQ ID NO: 14019 - protein, 9 aa, synthetic construct
GGLGGDHFV

SEQ ID NO: 14020 - protein, 9 aa, synthetic construct
GGVGNDIMI

SEQ ID NO: 14021 - protein, 9 aa, synthetic construct
GGGGSDTFM

SEQ ID NO: 14022 - protein, 9 aa, synthetic construct
GGEGFDTLS

SEQ ID NO: 14023 - protein, 9 aa, synthetic construct
GGGGDDDLN

SEQ ID NO: 14024 - protein, 9 aa, synthetic construct
GGAGKDELH

SEQ ID NO: 14025 - protein, 9 aa, synthetic construct
GGDGADSVE

SEQ ID NO: 14026 - protein, 9 aa, synthetic construct
GGQGDDLIL

SEQ ID NO: 14027 - protein, 9 aa, synthetic construct
GGDGDDVVY

SEQ ID NO: 14028 - protein, 9 aa, synthetic construct
GGEGADEFV

SEQ ID NO: 14029 - protein, 9 aa, synthetic construct
GGGGRDRID

SEQ ID NO: 14030 - protein, 9 aa, synthetic construct
GGSGRDFLD

SEQ ID NO: 14031 - protein, 9 aa, synthetic construct
GGGGDDDLE

SEQ ID NO: 14032 - protein, 9 aa, synthetic construct
GGNGPDIVL

SEQ ID NO: 14033 - protein, 9 aa, synthetic construct
GGVGNDEMY

SEQ ID NO: 14034 - protein, 9 aa, synthetic construct
GGLGGDDLW

SEQ ID NO: 14035 - protein, 9 aa, synthetic construct
GGNGMDTLW

SEQ ID NO: 14036 - protein, 9 aa, synthetic construct
GGNGDDSLN

SEQ ID NO: 14037 - protein, 9 aa, synthetic construct
GGLGNDVMK

SEQ ID NO: 14038 - protein, 9 aa, synthetic construct
GGGGNDRFY

SEQ ID NO: 14039 - protein, 9 aa, synthetic construct
GGQGDDFLS

SEQ ID NO: 14040 - protein, 9 aa, synthetic construct
GGGGKDDLR

SEQ ID NO: 14041 - protein, 9 aa, synthetic construct
GGGGRDRIE

SEQ ID NO: 14042 - protein, 9 aa, synthetic construct
GGAGTDDLR

SEQ ID NO: 14043 - protein, 9 aa, synthetic construct
GGNGMDTLQ

SEQ ID NO: 14044 - protein, 9 aa, synthetic construct
GGSGRDRML

SEQ ID NO: 14045 - protein, 9 aa, synthetic construct
GGEGFDVVT

SEQ ID NO: 14046 - protein, 9 aa, synthetic construct
GGGGSDSVT

SEQ ID NO: 14047 - protein, 9 aa, synthetic construct
GGDGHDILI

SEQ ID NO: 14048 - protein, 9 aa, synthetic construct
GGAGSDYLN

SEQ ID NO: 14049 - protein, 9 aa, synthetic construct
GGVGNDELQ

SEQ ID NO: 14050 - protein, 9 aa, synthetic construct
GGQGDDFLD

SEQ ID NO: 14051 - protein, 9 aa, synthetic construct
GGSGNDQVL

SEQ ID NO: 14052 - protein, 9 aa, synthetic construct
GGLGFDTLI

SEQ ID NO: 14053 - protein, 9 aa, synthetic construct
GGMGADTMI

SEQ ID NO: 14054 - protein, 9 aa, synthetic construct
GGGGSDSLD

SEQ ID NO: 14055 - protein, 9 aa, synthetic construct
GGMGADMLN

SEQ ID NO: 14056 - protein, 9 aa, synthetic construct
GGQGDDSLY

SEQ ID NO: 14057 - protein, 9 aa, synthetic construct
GGAGSDVVF

SEQ ID NO: 14058 - protein, 9 aa, synthetic construct
GGQGADRLI

SEQ ID NO: 14059 - protein, 9 aa, synthetic construct
GGNGRDKLL

SEQ ID NO: 14060 - protein, 9 aa, synthetic construct
GGQGDDSAS

SEQ ID NO: 14061 - protein, 9 aa, synthetic construct
GGEGDDFLI

SEQ ID NO: 14062 - protein, 9 aa, synthetic construct
GGDGKDVIR

SEQ ID NO: 14063 - protein, 9 aa, synthetic construct
GGNGRDKLY

SEQ ID NO: 14064 - protein, 9 aa, synthetic construct
GGAGSDVVI

SEQ ID NO: 14065 - protein, 9 aa, synthetic construct
GGGGHDELD

SEQ ID NO: 14066 - protein, 9 aa, synthetic construct
GGVGNDRIF

SEQ ID NO: 14067 - protein, 9 aa, synthetic construct
GGAGADFMH

SEQ ID NO: 14068 - protein, 9 aa, synthetic construct
GGGGRDQLS

SEQ ID NO: 14069 - protein, 9 aa, synthetic construct
GGQGDDRVF

SEQ ID NO: 14070 - protein, 9 aa, synthetic construct
GGEGKDTVE

SEQ ID NO: 14071 - protein, 9 aa, synthetic construct
GGQGADRFV

SEQ ID NO: 14072 - protein, 9 aa, synthetic construct
GGDGNDVVK

SEQ ID NO: 14073 - protein, 9 aa, synthetic construct
GGVGNDRIT

SEQ ID NO: 14074 - protein, 9 aa, synthetic construct
GGNGNDEIW

SEQ ID NO: 14075 - protein, 9 aa, synthetic construct
GGGGSDTVF

SEQ ID NO: 14076 - protein, 9 aa, synthetic construct
GGSGRDKLN

SEQ ID NO: 14077 - protein, 9 aa, synthetic construct
GGAGDDELE

SEQ ID NO: 14078 - protein, 9 aa, synthetic construct
GGEGSDFLN

SEQ ID NO: 14079 - protein, 9 aa, synthetic construct
GGEGNDDIS

SEQ ID NO: 14080 - protein, 9 aa, synthetic construct
GGHGHDWLR

SEQ ID NO: 14081 - protein, 9 aa, synthetic construct
GGVGNDRFF

SEQ ID NO: 14082 - protein, 9 aa, synthetic construct
GGGGGDLLT

SEQ ID NO: 14083 - protein, 9 aa, synthetic construct
GGQGDDRLN

SEQ ID NO: 14084 - protein, 9 aa, synthetic construct
GGAGKDVMT

SEQ ID NO: 14085 - protein, 9 aa, synthetic construct
GGGGIDTID

SEQ ID NO: 14086 - protein, 9 aa, synthetic construct
GGDGDDLLW

SEQ ID NO: 14087 - protein, 9 aa, synthetic construct
GGEGNDVIV

SEQ ID NO: 14088 - protein, 9 aa, synthetic construct
GGVGLDTLT

SEQ ID NO: 14089 - protein, 9 aa, synthetic construct
GGAGTDKLV

SEQ ID NO: 14090 - protein, 9 aa, synthetic construct
GGAGKDFLK

SEQ ID NO: 14091 - protein, 9 aa, synthetic construct
GGMGADLMT

SEQ ID NO: 14092 - protein, 9 aa, synthetic construct
GGQGADSIA

SEQ ID NO: 14093 - protein, 9 aa, synthetic construct
GGFGKDTLN

SEQ ID NO: 14094 - protein, 9 aa, synthetic construct
GGQGADRYL

SEQ ID NO: 14095 - protein, 9 aa, synthetic construct
GGMGNDSVY

SEQ ID NO: 14096 - protein, 9 aa, synthetic construct
GGYGNDQLH

SEQ ID NO: 14097 - protein, 9 aa, synthetic construct
GGQGDDRLS

SEQ ID NO: 14098 - protein, 9 aa, synthetic construct
GGDGEDSIS

SEQ ID NO: 14099 - protein, 9 aa, synthetic construct
GGEGRDDMY

SEQ ID NO: 14100 - protein, 9 aa, synthetic construct
GGEGNDTYF

SEQ ID NO: 14101 - protein, 9 aa, synthetic construct
GGQGADRLY

SEQ ID NO: 14102 - protein, 9 aa, synthetic construct
GGNGLDVLV

SEQ ID NO: 14103 - protein, 9 aa, synthetic construct
GGVGNDQMW

SEQ ID NO: 14104 - protein, 9 aa, synthetic construct
GGLGGDVFR

SEQ ID NO: 14105 - protein, 9 aa, synthetic construct
GGAGTDLAN

SEQ ID NO: 14106 - protein, 9 aa, synthetic construct
GGNGRDLIY

SEQ ID NO: 14107 - protein, 9 aa, synthetic construct
GGGGDDFLL

SEQ ID NO: 14108 - protein, 9 aa, synthetic construct
GGLGGDVLI

SEQ ID NO: 14109 - protein, 9 aa, synthetic construct
GGQGADLLD

SEQ ID NO: 14110 - protein, 9 aa, synthetic construct
GGSGNDRMW

SEQ ID NO: 14111 - protein, 9 aa, synthetic construct
GGFGLDVLD

SEQ ID NO: 14112 - protein, 9 aa, synthetic construct
GGNGNDELN

SEQ ID NO: 14113 - protein, 9 aa, synthetic construct
GGGGSDTVS

SEQ ID NO: 14114 - protein, 9 aa, synthetic construct
GGHGKDQIF

SEQ ID NO: 14115 - protein, 9 aa, synthetic construct
GGGGSDRLQ

SEQ ID NO: 14116 - protein, 9 aa, synthetic construct
GGEGLDTLL

SEQ ID NO: 14117 - protein, 9 aa, synthetic construct
GGNGRDLVY

SEQ ID NO: 14118 - protein, 9 aa, synthetic construct
GGQGADLLK

SEQ ID NO: 14119 - protein, 9 aa, synthetic construct
GGEGNDTVY

SEQ ID NO: 14120 - protein, 9 aa, synthetic construct
GGKGDDILE

SEQ ID NO: 14121 - protein, 9 aa, synthetic construct
GGSGNDRME

SEQ ID NO: 14122 - protein, 9 aa, synthetic construct
GGGGNDRLG

SEQ ID NO: 14123 - protein, 9 aa, synthetic construct
GGNGNDTMY

SEQ ID NO: 14124 - protein, 9 aa, synthetic construct
GGDGDDVVL

SEQ ID NO: 14125 - protein, 9 aa, synthetic construct
GGEGNDDIG

SEQ ID NO: 14126 - protein, 9 aa, synthetic construct
GGGGLDVMH

SEQ ID NO: 14127 - protein, 9 aa, synthetic construct
GGAGADFVA

SEQ ID NO: 14128 - protein, 9 aa, synthetic construct
GGLGGDYLI

SEQ ID NO: 14129 - protein, 9 aa, synthetic construct
GGAGTDLVK

SEQ ID NO: 14130 - protein, 9 aa, synthetic construct
GGSGNDRVI

SEQ ID NO: 14131 - protein, 9 aa, synthetic construct
GGAGTDLVL

SEQ ID NO: 14132 - protein, 9 aa, synthetic construct
GGAGDDHIL

SEQ ID NO: 14133 - protein, 9 aa, synthetic construct
GGEGQDTFR

SEQ ID NO: 14134 - protein, 9 aa, synthetic construct
GGQGDDSLF

SEQ ID NO: 14135 - protein, 9 aa, synthetic construct
GGAGMDALD

SEQ ID NO: 14136 - protein, 9 aa, synthetic construct
GGDGDDALI

SEQ ID NO: 14137 - protein, 9 aa, synthetic construct
GGHGIDQID

SEQ ID NO: 14138 - protein, 9 aa, synthetic construct
GGAGKDHFV

SEQ ID NO: 14139 - protein, 9 aa, synthetic construct
GGMGADLLT

SEQ ID NO: 14140 - protein, 9 aa, synthetic construct
GGQGADNLF

SEQ ID NO: 14141 - protein, 9 aa, synthetic construct
GGNGRDLLF

SEQ ID NO: 14142 - protein, 9 aa, synthetic construct
GGQGDDSIQ

SEQ ID NO: 14143 - protein, 9 aa, synthetic construct
GGDGADRIW

SEQ ID NO: 14144 - protein, 9 aa, synthetic construct
GGNGDDSLW

SEQ ID NO: 14145 - protein, 9 aa, synthetic construct
GGKGADQVW

SEQ ID NO: 14146 - protein, 9 aa, synthetic construct
GGEGSDIYI

SEQ ID NO: 14147 - protein, 9 aa, synthetic construct
GGQGADLVM

SEQ ID NO: 14148 - protein, 9 aa, synthetic construct
GGDGADRIT

SEQ ID NO: 14149 - protein, 9 aa, synthetic construct
GGNGDDMLI

SEQ ID NO: 14150 - protein, 9 aa, synthetic construct
GGQGADLMR

SEQ ID NO: 14151 - protein, 9 aa, synthetic construct
GGSGTDTFQ

SEQ ID NO: 14152 - protein, 9 aa, synthetic construct
GGNGRDLLV

SEQ ID NO: 14153 - protein, 9 aa, synthetic construct
GGLGNDTYA

SEQ ID NO: 14154 - protein, 9 aa, synthetic construct
GGSGRDRAL

SEQ ID NO: 14155 - protein, 9 aa, synthetic construct
GGDGKDKLK

SEQ ID NO: 14156 - protein, 9 aa, synthetic construct
GGLGNDTVY

SEQ ID NO: 14157 - protein, 9 aa, synthetic construct
GGLGVDNLT

SEQ ID NO: 14158 - protein, 9 aa, synthetic construct
GGGGSDKLL

SEQ ID NO: 14159 - protein, 9 aa, synthetic construct
GGNGRDILI

SEQ ID NO: 14160 - protein, 9 aa, synthetic construct
GGAGSDWLI

SEQ ID NO: 14161 - protein, 9 aa, synthetic construct
GGNGQDTLY

SEQ ID NO: 14162 - protein, 9 aa, synthetic construct
GGDGKDLLY

SEQ ID NO: 14163 - protein, 9 aa, synthetic construct
GGKGADQLA

SEQ ID NO: 14164 - protein, 9 aa, synthetic construct
GGQGADTLY

SEQ ID NO: 14165 - protein, 9 aa, synthetic construct
GGKGDDLIF

SEQ ID NO: 14166 - protein, 9 aa, synthetic construct
GGNGDDLVY

SEQ ID NO: 14167 - protein, 9 aa, synthetic construct
GGHGDDYLD

SEQ ID NO: 14168 - protein, 9 aa, synthetic construct
GGNGNDSLW

SEQ ID NO: 14169 - protein, 9 aa, synthetic construct
GGEGDDWIE

SEQ ID NO: 14170 - protein, 9 aa, synthetic construct
GGLGNDVIF

SEQ ID NO: 14171 - protein, 9 aa, synthetic construct
GGGGNDSFE

SEQ ID NO: 14172 - protein, 9 aa, synthetic construct
GGKGEDVLF

SEQ ID NO: 14173 - protein, 9 aa, synthetic construct
GGLGNDVIE

SEQ ID NO: 14174 - protein, 9 aa, synthetic construct
GGEGQDTLN

SEQ ID NO: 14175 - protein, 9 aa, synthetic construct
GGYGNDSLV

SEQ ID NO: 14176 - protein, 9 aa, synthetic construct
GGGGIDYLA

SEQ ID NO: 14177 - protein, 9 aa, synthetic construct
GGLGGDTID

SEQ ID NO: 14178 - protein, 9 aa, synthetic construct
GGYGNDSLR

SEQ ID NO: 14179 - protein, 9 aa, synthetic construct
GGLGRDALF

SEQ ID NO: 14180 - protein, 9 aa, synthetic construct
GGGGHDELL

SEQ ID NO: 14181 - protein, 9 aa, synthetic construct
GGGGSDLLE

SEQ ID NO: 14182 - protein, 9 aa, synthetic construct
GGLGGDTIF

SEQ ID NO: 14183 - protein, 9 aa, synthetic construct
GGSGRDILN

SEQ ID NO: 14184 - protein, 9 aa, synthetic construct
GGDGNDVVF

SEQ ID NO: 14185 - protein, 9 aa, synthetic construct
GGVGNDLVD

SEQ ID NO: 14186 - protein, 9 aa, synthetic construct
GGLGNDVII

SEQ ID NO: 14187 - protein, 9 aa, synthetic construct
GGGGDDELR

SEQ ID NO: 14188 - protein, 9 aa, synthetic construct
GGQGDDMLW

SEQ ID NO: 14189 - protein, 9 aa, synthetic construct
GGAGTDIIE

SEQ ID NO: 14190 - protein, 9 aa, synthetic construct
GGEGFDTFI

SEQ ID NO: 14191 - protein, 9 aa, synthetic construct
GGGGDDELT

SEQ ID NO: 14192 - protein, 9 aa, synthetic construct
GGQGDDMLY

SEQ ID NO: 14193 - protein, 9 aa, synthetic construct
GGLGNDWLQ

SEQ ID NO: 14194 - protein, 9 aa, synthetic construct
GGAGSDWLY

SEQ ID NO: 14195 - protein, 9 aa, synthetic construct
GGAGADFFF

SEQ ID NO: 14196 - protein, 9 aa, synthetic construct
GGDGADSIA

SEQ ID NO: 14197 - protein, 9 aa, synthetic construct
GGDGNDVMV

SEQ ID NO: 14198 - protein, 9 aa, synthetic construct
GGQGADTMY

SEQ ID NO: 14199 - protein, 9 aa, synthetic construct
GGAGSDWLW

SEQ ID NO: 14200 - protein, 9 aa, synthetic construct
GGVGNDLMT

SEQ ID NO: 14201 - protein, 9 aa, synthetic construct
GGEGQDTLS

SEQ ID NO: 14202 - protein, 9 aa, synthetic construct
GGAGSDWLT

SEQ ID NO: 14203 - protein, 9 aa, synthetic construct
GGAGDDGLD

SEQ ID NO: 14204 - protein, 9 aa, synthetic construct
GGQGADTMR

SEQ ID NO: 14205 - protein, 9 aa, synthetic construct
GGSGRDEIR

SEQ ID NO: 14206 - protein, 9 aa, synthetic construct
GGGGDDELV

SEQ ID NO: 14207 - protein, 9 aa, synthetic construct
GGYGSDEIY

SEQ ID NO: 14208 - protein, 9 aa, synthetic construct
GGDGHDFLN

SEQ ID NO: 14209 - protein, 9 aa, synthetic construct
GGKGEDLLK

SEQ ID NO: 14210 - protein, 9 aa, synthetic construct
GGQGADSLA

SEQ ID NO: 14211 - protein, 9 aa, synthetic construct
GGQGADSLS

SEQ ID NO: 14212 - protein, 9 aa, synthetic construct
GGNGRDFIF

SEQ ID NO: 14213 - protein, 9 aa, synthetic construct
GGQGDDRAF

SEQ ID NO: 14214 - protein, 9 aa, synthetic construct
GGNGNDVFA

SEQ ID NO: 14215 - protein, 9 aa, synthetic construct
GGLGNDVAV

SEQ ID NO: 14216 - protein, 9 aa, synthetic construct
GGAGADFID

SEQ ID NO: 14217 - protein, 9 aa, synthetic construct
GGAGADFIF

SEQ ID NO: 14218 - protein, 9 aa, synthetic construct
GGAGSDVYV

SEQ ID NO: 14219 - protein, 9 aa, synthetic construct
GGAGKDFIY

SEQ ID NO: 14220 - protein, 9 aa, synthetic construct
GGLGNDTYW

SEQ ID NO: 14221 - protein, 9 aa, synthetic construct
GGYGNDRLT

SEQ ID NO: 14222 - protein, 9 aa, synthetic construct
GGAGDDGLS

SEQ ID NO: 14223 - protein, 9 aa, synthetic construct
GGDGKDLLR

SEQ ID NO: 14224 - protein, 9 aa, synthetic construct
GGAGADDIA

SEQ ID NO: 14225 - protein, 9 aa, synthetic construct
GGKGDDILL

SEQ ID NO: 14226 - protein, 9 aa, synthetic construct
GGEGNDDMR

SEQ ID NO: 14227 - protein, 9 aa, synthetic construct
GGEGNDVIS

SEQ ID NO: 14228 - protein, 9 aa, synthetic construct
GGAGSDVYN

SEQ ID NO: 14229 - protein, 9 aa, synthetic construct
GGDGADYMQ

SEQ ID NO: 14230 - protein, 9 aa, synthetic construct
GGYGNDRIY

SEQ ID NO: 14231 - protein, 9 aa, synthetic construct
GGQGADSLF

SEQ ID NO: 14232 - protein, 9 aa, synthetic construct
GGHGHDTVR

SEQ ID NO: 14233 - protein, 9 aa, synthetic construct
GGEGNDDIY

SEQ ID NO: 14234 - protein, 9 aa, synthetic construct
GGVGNDNLY

SEQ ID NO: 14235 - protein, 9 aa, synthetic construct
GGDGADRMS

SEQ ID NO: 14236 - protein, 9 aa, synthetic construct
GGGGNDALV

SEQ ID NO: 14237 - protein, 9 aa, synthetic construct
GGNGRDELR

SEQ ID NO: 14238 - protein, 9 aa, synthetic construct
GGHGDDVLT

SEQ ID NO: 14239 - protein, 9 aa, synthetic construct
GGQGADTLE

SEQ ID NO: 14240 - protein, 9 aa, synthetic construct
GGEGFDYLA

SEQ ID NO: 14241 - protein, 9 aa, synthetic construct
GGSGTDLLI

SEQ ID NO: 14242 - protein, 9 aa, synthetic construct
GGNGRDALD

SEQ ID NO: 14243 - protein, 9 aa, synthetic construct
GGDGPDRLF

SEQ ID NO: 14244 - protein, 9 aa, synthetic construct
GGGGSDLLI

SEQ ID NO: 14245 - protein, 9 aa, synthetic construct
GGMGADTLD

SEQ ID NO: 14246 - protein, 9 aa, synthetic construct
GGMGNDLMI

SEQ ID NO: 14247 - protein, 9 aa, synthetic construct
GGEGKDTMN

SEQ ID NO: 14248 - protein, 9 aa, synthetic construct
GGNGNDVFY

SEQ ID NO: 14249 - protein, 9 aa, synthetic construct
GGDGKDTLV

SEQ ID NO: 14250 - protein, 9 aa, synthetic construct
GGAGADDIG

SEQ ID NO: 14251 - protein, 9 aa, synthetic construct
GGDGNDVYR

SEQ ID NO: 14252 - protein, 9 aa, synthetic construct
GGDGNDVMN

SEQ ID NO: 14253 - protein, 9 aa, synthetic construct
GGAGDDEVY

SEQ ID NO: 14254 - protein, 9 aa, synthetic construct
GGGGGDTLL

SEQ ID NO: 14255 - protein, 9 aa, synthetic construct
GGYGNDSID

SEQ ID NO: 14256 - protein, 9 aa, synthetic construct
GGFGNDPIP

SEQ ID NO: 14257 - protein, 9 aa, synthetic construct
GGNGNDVFD

SEQ ID NO: 14258 - protein, 9 aa, synthetic construct
GGGGRDRLY

SEQ ID NO: 14259 - protein, 9 aa, synthetic construct
GGLGGDKLF

SEQ ID NO: 14260 - protein, 9 aa, synthetic construct
GGGGVDLLK

SEQ ID NO: 14261 - protein, 9 aa, synthetic construct
GGEGSDEID

SEQ ID NO: 14262 - protein, 9 aa, synthetic construct
GGSGSDNLN

SEQ ID NO: 14263 - protein, 9 aa, synthetic construct
GGLGNDALK

SEQ ID NO: 14264 - protein, 9 aa, synthetic construct
GGLGNDALI

SEQ ID NO: 14265 - protein, 9 aa, synthetic construct
GGDGADALS

SEQ ID NO: 14266 - protein, 9 aa, synthetic construct
GGLGNDALH

SEQ ID NO: 14267 - protein, 9 aa, synthetic construct
GGDGADALT

SEQ ID NO: 14268 - protein, 9 aa, synthetic construct
GGGGTDTLE

SEQ ID NO: 14269 - protein, 9 aa, synthetic construct
GGGGDDQIR

SEQ ID NO: 14270 - protein, 9 aa, synthetic construct
GGAGADLMY

SEQ ID NO: 14271 - protein, 9 aa, synthetic construct
GGDGVDTIL

SEQ ID NO: 14272 - protein, 9 aa, synthetic construct
GGDGADALW

SEQ ID NO: 14273 - protein, 9 aa, synthetic construct
GGLGNDALD

SEQ ID NO: 14274 - protein, 9 aa, synthetic construct
GGAGVDTAN

SEQ ID NO: 14275 - protein, 9 aa, synthetic construct
GGAGADLVY

SEQ ID NO: 14276 - protein, 9 aa, synthetic construct
GGLGNDALA

SEQ ID NO: 14277 - protein, 9 aa, synthetic construct
GGGGDDQLD

SEQ ID NO: 14278 - protein, 9 aa, synthetic construct
GGAGKDSLF

SEQ ID NO: 14279 - protein, 9 aa, synthetic construct
GGKGADVFR

SEQ ID NO: 14280 - protein, 9 aa, synthetic construct
GGAGVDTFM

SEQ ID NO: 14281 - protein, 9 aa, synthetic construct
GGPGHDTLY

SEQ ID NO: 14282 - protein, 9 aa, synthetic construct
GGNGNDLIL

SEQ ID NO: 14283 - protein, 9 aa, synthetic construct
GGAGADLYV

SEQ ID NO: 14284 - protein, 9 aa, synthetic construct
GGSGSDMLN

SEQ ID NO: 14285 - protein, 9 aa, synthetic construct
GGSGSDELN

SEQ ID NO: 14286 - protein, 9 aa, synthetic construct
GGDGHDRIT

SEQ ID NO: 14287 - protein, 9 aa, synthetic construct
GGLGNDNFR

SEQ ID NO: 14288 - protein, 9 aa, synthetic construct
GGWGDDIVD

SEQ ID NO: 14289 - protein, 9 aa, synthetic construct
GGGGTDTLK

SEQ ID NO: 14290 - protein, 9 aa, synthetic construct
GGPGHDTIY

SEQ ID NO: 14291 - protein, 9 aa, synthetic construct
GGGGDDVAL

SEQ ID NO: 14292 - protein, 9 aa, synthetic construct
GGDGADVIE

SEQ ID NO: 14293 - protein, 9 aa, synthetic construct
GGAGKDQFI

SEQ ID NO: 14294 - protein, 9 aa, synthetic construct
GGGGKDRLI

SEQ ID NO: 14295 - protein, 9 aa, synthetic construct
GGDGEDALS

SEQ ID NO: 14296 - protein, 9 aa, synthetic construct
GGAGVDTAF

SEQ ID NO: 14297 - protein, 9 aa, synthetic construct
GGKGDDVLK

SEQ ID NO: 14298 - protein, 9 aa, synthetic construct
GGPGADILI

SEQ ID NO: 14299 - protein, 9 aa, synthetic construct
GGYGADTVM

SEQ ID NO: 14300 - protein, 9 aa, synthetic construct
GGPGADILS

SEQ ID NO: 14301 - protein, 9 aa, synthetic construct
GGAGADLVD

SEQ ID NO: 14302 - protein, 9 aa, synthetic construct
GGAGLDQLN

SEQ ID NO: 14303 - protein, 9 aa, synthetic construct
GGEGNDALG

SEQ ID NO: 14304 - protein, 9 aa, synthetic construct
GGAGVDSLL

SEQ ID NO: 14305 - protein, 9 aa, synthetic construct
GGPGADILY

SEQ ID NO: 14306 - protein, 9 aa, synthetic construct
GGAGADTVG

SEQ ID NO: 14307 - protein, 9 aa, synthetic construct
GGAGKDMFV

SEQ ID NO: 14308 - protein, 9 aa, synthetic construct
GGAGVDSLV

SEQ ID NO: 14309 - protein, 9 aa, synthetic construct
GGPGIDTLV

SEQ ID NO: 14310 - protein, 9 aa, synthetic construct
GGSGNDVIF

SEQ ID NO: 14311 - protein, 9 aa, synthetic construct
GGAGLDQLQ

SEQ ID NO: 14312 - protein, 9 aa, synthetic construct
GGGGTDTLD

SEQ ID NO: 14313 - protein, 9 aa, synthetic construct
GGLGSDQLF

SEQ ID NO: 14314 - protein, 9 aa, synthetic construct
GGKGADVFA

SEQ ID NO: 14315 - protein, 9 aa, synthetic construct
GGPGADKLF

SEQ ID NO: 14316 - protein, 9 aa, synthetic construct
GGPGIDTAV

SEQ ID NO: 14317 - protein, 9 aa, synthetic construct
GGNGDDTFI

SEQ ID NO: 14318 - protein, 9 aa, synthetic construct
GGGGDDQAV

SEQ ID NO: 14319 - protein, 9 aa, synthetic construct
GGLGNDAFV

SEQ ID NO: 14320 - protein, 9 aa, synthetic construct
GGLGNDAID

SEQ ID NO: 14321 - protein, 9 aa, synthetic construct
GGLGNDNIT

SEQ ID NO: 14322 - protein, 9 aa, synthetic construct
GGDGNDYLH

SEQ ID NO: 14323 - protein, 9 aa, synthetic construct
GGGGKDRLN

SEQ ID NO: 14324 - protein, 9 aa, synthetic construct
GGGGDDVFI

SEQ ID NO: 14325 - protein, 9 aa, synthetic construct
GGGGKDKLW

SEQ ID NO: 14326 - protein, 9 aa, synthetic construct
GGPGADLFV

SEQ ID NO: 14327 - protein, 9 aa, synthetic construct
GGPGADLID

SEQ ID NO: 14328 - protein, 9 aa, synthetic construct
GGWGDDLLD

SEQ ID NO: 14329 - protein, 9 aa, synthetic construct
GGGGDDTYY

SEQ ID NO: 14330 - protein, 9 aa, synthetic construct
GGAGKDSLD

SEQ ID NO: 14331 - protein, 9 aa, synthetic construct
GGGGTDTMY

SEQ ID NO: 14332 - protein, 9 aa, synthetic construct
GGCGNDNIQ

SEQ ID NO: 14333 - protein, 9 aa, synthetic construct
GGAGVDTMA

SEQ ID NO: 14334 - protein, 9 aa, synthetic construct
GGDGVDTLF

SEQ ID NO: 14335 - protein, 9 aa, synthetic construct
GGGGKDLLD

SEQ ID NO: 14336 - protein, 9 aa, synthetic construct
GGLGNDDLD

SEQ ID NO: 14337 - protein, 9 aa, synthetic construct
GGPGADRML

SEQ ID NO: 14338 - protein, 9 aa, synthetic construct
GGAGADTAV

SEQ ID NO: 14339 - protein, 9 aa, synthetic construct
GGDGVDTLG

SEQ ID NO: 14340 - protein, 9 aa, synthetic construct
GGDGADVIG

SEQ ID NO: 14341 - protein, 9 aa, synthetic construct
GGPGGDTLV

SEQ ID NO: 14342 - protein, 9 aa, synthetic construct
GGGGDDTVL

SEQ ID NO: 14343 - protein, 9 aa, synthetic construct
GGGGDDTVI

SEQ ID NO: 14344 - protein, 9 aa, synthetic construct
GGPGGDTLT

SEQ ID NO: 14345 - protein, 9 aa, synthetic construct
GGAGADMIT

SEQ ID NO: 14346 - protein, 9 aa, synthetic construct
GGPGADSLA

SEQ ID NO: 14347 - protein, 9 aa, synthetic construct
GGWGDDTFI

SEQ ID NO: 14348 - protein, 9 aa, synthetic construct
GGEGRDTFL

SEQ ID NO: 14349 - protein, 9 aa, synthetic construct
GGEGKDVLD

SEQ ID NO: 14350 - protein, 9 aa, synthetic construct
GGSGNDVMD

SEQ ID NO: 14351 - protein, 9 aa, synthetic construct
GGGGTDTVD

SEQ ID NO: 14352 - protein, 9 aa, synthetic construct
GGYGADQLT

SEQ ID NO: 14353 - protein, 9 aa, synthetic construct
GGWGDDTLY

SEQ ID NO: 14354 - protein, 9 aa, synthetic construct
GGPGADSLI

SEQ ID NO: 14355 - protein, 9 aa, synthetic construct
GGNGDDRLL

SEQ ID NO: 14356 - protein, 9 aa, synthetic construct
GGPGGDSLS

SEQ ID NO: 14357 - protein, 9 aa, synthetic construct
GGAGADSYV

SEQ ID NO: 14358 - protein, 9 aa, synthetic construct
GGLGNDDLS

SEQ ID NO: 14359 - protein, 9 aa, synthetic construct
GGPGADSLV

SEQ ID NO: 14360 - protein, 9 aa, synthetic construct
GGGGDDTVE

SEQ ID NO: 14361 - protein, 9 aa, synthetic construct
GGAGADSYD

SEQ ID NO: 14362 - protein, 9 aa, synthetic construct
GGGGVDYVW

SEQ ID NO: 14363 - protein, 9 aa, synthetic construct
GGLGNDMLL

SEQ ID NO: 14364 - protein, 9 aa, synthetic construct
GGDGEDVVN

SEQ ID NO: 14365 - protein, 9 aa, synthetic construct
GGLGNDAYV

SEQ ID NO: 14366 - protein, 9 aa, synthetic construct
GGGGKDKLY

SEQ ID NO: 14367 - protein, 9 aa, synthetic construct
GGDGHDRLA

SEQ ID NO: 14368 - protein, 9 aa, synthetic construct
GGPGHDRLI

SEQ ID NO: 14369 - protein, 9 aa, synthetic construct
GGDGADAID

SEQ ID NO: 14370 - protein, 9 aa, synthetic construct
GGWGDDNLL

SEQ ID NO: 14371 - protein, 9 aa, synthetic construct
GGLGNDAVN

SEQ ID NO: 14372 - protein, 9 aa, synthetic construct
GGLGNDAVV

SEQ ID NO: 14373 - protein, 9 aa, synthetic construct
GGAGVDTIS

SEQ ID NO: 14374 - protein, 9 aa, synthetic construct
GGPGADQLV

SEQ ID NO: 14375 - protein, 9 aa, synthetic construct
GGAGADTFW

SEQ ID NO: 14376 - protein, 9 aa, synthetic construct
GGSGSDELW

SEQ ID NO: 14377 - protein, 9 aa, synthetic construct
GGWGDDQLW

SEQ ID NO: 14378 - protein, 9 aa, synthetic construct
GGPGHDMLR

SEQ ID NO: 14379 - protein, 9 aa, synthetic construct
GGNGNDLIS

SEQ ID NO: 14380 - protein, 9 aa, synthetic construct
GGLGNDMLR

SEQ ID NO: 14381 - protein, 9 aa, synthetic construct
GGEGRDLVS

SEQ ID NO: 14382 - protein, 9 aa, synthetic construct
GGKGADVLI

SEQ ID NO: 14383 - protein, 9 aa, synthetic construct
GGAGADMID

SEQ ID NO: 14384 - protein, 9 aa, synthetic construct
GGEGNDALA

SEQ ID NO: 14385 - protein, 9 aa, synthetic construct
GGNGNDQLL

SEQ ID NO: 14386 - protein, 9 aa, synthetic construct
GGPGADRFV

SEQ ID NO: 14387 - protein, 9 aa, synthetic construct
GGGGTDTLQ

SEQ ID NO: 14388 - protein, 9 aa, synthetic construct
GGEGDDRID

SEQ ID NO: 14389 - protein, 9 aa, synthetic construct
GGGGDDTVT

SEQ ID NO: 14390 - protein, 9 aa, synthetic construct
GGAGKDSLA

SEQ ID NO: 14391 - protein, 9 aa, synthetic construct
GGLGVDTVT

SEQ ID NO: 14392 - protein, 9 aa, synthetic construct
GGLGVDTVV

SEQ ID NO: 14393 - protein, 9 aa, synthetic construct
GGDGHDVLQ

SEQ ID NO: 14394 - protein, 9 aa, synthetic construct
GGPGADRLD

SEQ ID NO: 14395 - protein, 9 aa, synthetic construct
GGNGDDRLN

SEQ ID NO: 14396 - protein, 9 aa, synthetic construct
GGAGADTVH

SEQ ID NO: 14397 - protein, 9 aa, synthetic construct
GGAGVDSIY

SEQ ID NO: 14398 - protein, 9 aa, synthetic construct
GGLGNDQYI

SEQ ID NO: 14399 - protein, 9 aa, synthetic construct
GGEGNDYVS

SEQ ID NO: 14400 - protein, 9 aa, synthetic construct
GGDGVDSLL

SEQ ID NO: 14401 - protein, 9 aa, synthetic construct
GGPGNDELH

SEQ ID NO: 14402 - protein, 9 aa, synthetic construct
GGLGQDMLM

SEQ ID NO: 14403 - protein, 9 aa, synthetic construct
GGGGRDVLF

SEQ ID NO: 14404 - protein, 9 aa, synthetic construct
GGDGNDWLT

SEQ ID NO: 14405 - protein, 9 aa, synthetic construct
GGPGNDELR

SEQ ID NO: 14406 - protein, 9 aa, synthetic construct
GGGGKDTIL

SEQ ID NO: 14407 - protein, 9 aa, synthetic construct
GGAGADTVI

SEQ ID NO: 14408 - protein, 9 aa, synthetic construct
GGGGTDSLS

SEQ ID NO: 14409 - protein, 9 aa, synthetic construct
GGNGWDVLI

SEQ ID NO: 14410 - protein, 9 aa, synthetic construct
GGGGNDRIS

SEQ ID NO: 14411 - protein, 9 aa, synthetic construct
GGGGDDMLL

SEQ ID NO: 14412 - protein, 9 aa, synthetic construct
GGAGVDQLD

SEQ ID NO: 14413 - protein, 9 aa, synthetic construct
GGKGDDTAK

SEQ ID NO: 14414 - protein, 9 aa, synthetic construct
GGGGKDTIE

SEQ ID NO: 14415 - protein, 9 aa, synthetic construct
GGDGEDLVA

SEQ ID NO: 14416 - protein, 9 aa, synthetic construct
GGAGKDLLD

SEQ ID NO: 14417 - protein, 9 aa, synthetic construct
GGDGNDWLV

SEQ ID NO: 14418 - protein, 9 aa, synthetic construct
GGVGVDQYV

SEQ ID NO: 14419 - protein, 9 aa, synthetic construct
GGNGDDTAS

SEQ ID NO: 14420 - protein, 9 aa, synthetic construct
GGGGDDMLT

SEQ ID NO: 14421 - protein, 9 aa, synthetic construct
GGFGNDFVW

SEQ ID NO: 14422 - protein, 9 aa, synthetic construct
GGLGLDTLK

SEQ ID NO: 14423 - protein, 9 aa, synthetic construct
GGDGADEIS

SEQ ID NO: 14424 - protein, 9 aa, synthetic construct
GGDGDDLIW

SEQ ID NO: 14425 - protein, 9 aa, synthetic construct
GGLGLDTLN

SEQ ID NO: 14426 - protein, 9 aa, synthetic construct
GGAGVDRAV

SEQ ID NO: 14427 - protein, 9 aa, synthetic construct
GGNGNDRFF

SEQ ID NO: 14428 - protein, 9 aa, synthetic construct
GGDGADEIH

SEQ ID NO: 14429 - protein, 9 aa, synthetic construct
GGDGVDSLR

SEQ ID NO: 14430 - protein, 9 aa, synthetic construct
GGEGADIML

SEQ ID NO: 14431 - protein, 9 aa, synthetic construct
GGNGNDKLN

SEQ ID NO: 14432 - protein, 9 aa, synthetic construct
GGDGNDVIK

SEQ ID NO: 14433 - protein, 9 aa, synthetic construct
GGSGNDTYH

SEQ ID NO: 14434 - protein, 9 aa, synthetic construct
GGKGADTLQ

SEQ ID NO: 14435 - protein, 9 aa, synthetic construct
GGMGHDILD

SEQ ID NO: 14436 - protein, 9 aa, synthetic construct
GGFGNDFLE

SEQ ID NO: 14437 - protein, 9 aa, synthetic construct
GGLGNDQVN

SEQ ID NO: 14438 - protein, 9 aa, synthetic construct
GGDGADFIN

SEQ ID NO: 14439 - protein, 9 aa, synthetic construct
GGGGKDTLK

SEQ ID NO: 14440 - protein, 9 aa, synthetic construct
GGNGWDIIR

SEQ ID NO: 14441 - protein, 9 aa, synthetic construct
GGPGNDILD

SEQ ID NO: 14442 - protein, 9 aa, synthetic construct
GGDGDDYVE

SEQ ID NO: 14443 - protein, 9 aa, synthetic construct
GGPGNDIIN

SEQ ID NO: 14444 - protein, 9 aa, synthetic construct
GGPGNDIIE

SEQ ID NO: 14445 - protein, 9 aa, synthetic construct
GGAGKDSLI

SEQ ID NO: 14446 - protein, 9 aa, synthetic construct
GGNGNDKLA

SEQ ID NO: 14447 - protein, 9 aa, synthetic construct
GGEGDDRYV

SEQ ID NO: 14448 - protein, 9 aa, synthetic construct
GGPGNDIFI

SEQ ID NO: 14449 - protein, 9 aa, synthetic construct
GGLGLDRLV

SEQ ID NO: 14450 - protein, 9 aa, synthetic construct
GGYGDDILR

SEQ ID NO: 14451 - protein, 9 aa, synthetic construct
GGVGTDTLV

SEQ ID NO: 14452 - protein, 9 aa, synthetic construct
GGAGKDLIH

SEQ ID NO: 14453 - protein, 9 aa, synthetic construct
GGDGEDMLF

SEQ ID NO: 14454 - protein, 9 aa, synthetic construct
GGNGNDRIF

SEQ ID NO: 14455 - protein, 9 aa, synthetic construct
GGGGDDVLG

SEQ ID NO: 14456 - protein, 9 aa, synthetic construct
GGNGNDKLE

SEQ ID NO: 14457 - protein, 9 aa, synthetic construct
GGKGADTLR

SEQ ID NO: 14458 - protein, 9 aa, synthetic construct
GGNGNDRIE

SEQ ID NO: 14459 - protein, 9 aa, synthetic construct
GGAGADLIR

SEQ ID NO: 14460 - protein, 9 aa, synthetic construct
GGAGVDQFL

SEQ ID NO: 14461 - protein, 9 aa, synthetic construct
GGAGADVIK

SEQ ID NO: 14462 - protein, 9 aa, synthetic construct
GGSGQDFLN

SEQ ID NO: 14463 - protein, 9 aa, synthetic construct
GGLGLDTAT

SEQ ID NO: 14464 - protein, 9 aa, synthetic construct
GGYGDDILS

SEQ ID NO: 14465 - protein, 9 aa, synthetic construct
GGDGADEIG

SEQ ID NO: 14466 - protein, 9 aa, synthetic construct
GGKGADTLW

SEQ ID NO: 14467 - protein, 9 aa, synthetic construct
GGPGNDAIS

SEQ ID NO: 14468 - protein, 9 aa, synthetic construct
GGGGDDVFT

SEQ ID NO: 14469 - protein, 9 aa, synthetic construct
GGPGKDVLT

SEQ ID NO: 14470 - protein, 9 aa, synthetic construct
GGDGADDLR

SEQ ID NO: 14471 - protein, 9 aa, synthetic construct
GGSGNDVFI

SEQ ID NO: 14472 - protein, 9 aa, synthetic construct
GGPGKDVIY

SEQ ID NO: 14473 - protein, 9 aa, synthetic construct
GGGGDDVFY

SEQ ID NO: 14474 - protein, 9 aa, synthetic construct
GGDGEDAFV

SEQ ID NO: 14475 - protein, 9 aa, synthetic construct
GGLGNDQIF

SEQ ID NO: 14476 - protein, 9 aa, synthetic construct
GGLGQDKLY

SEQ ID NO: 14477 - protein, 9 aa, synthetic construct
GGEGEDTIS

SEQ ID NO: 14478 - protein, 9 aa, synthetic construct
GGGGTDTID

SEQ ID NO: 14479 - protein, 9 aa, synthetic construct
GGEGEDTIL

SEQ ID NO: 14480 - protein, 9 aa, synthetic construct
GGAGVDSAN

SEQ ID NO: 14481 - protein, 9 aa, synthetic construct
GGAGVDSAS

SEQ ID NO: 14482 - protein, 9 aa, synthetic construct
GGGGDDNLH

SEQ ID NO: 14483 - protein, 9 aa, synthetic construct
GGGGTDTIN

SEQ ID NO: 14484 - protein, 9 aa, synthetic construct
GGGGDDNIS

SEQ ID NO: 14485 - protein, 9 aa, synthetic construct
GGAGVDSFG

SEQ ID NO: 14486 - protein, 9 aa, synthetic construct
GGEGNDALK

SEQ ID NO: 14487 - protein, 9 aa, synthetic construct
GGPGKDTLD

SEQ ID NO: 14488 - protein, 9 aa, synthetic construct
GGAGVDSFT

SEQ ID NO: 14489 - protein, 9 aa, synthetic construct
GGWGADHME

SEQ ID NO: 14490 - protein, 9 aa, synthetic construct
GGAGLDTLF

SEQ ID NO: 14491 - protein, 9 aa, synthetic construct
GGDGADVMS

SEQ ID NO: 14492 - protein, 9 aa, synthetic construct
GGWGADHMQ

SEQ ID NO: 14493 - protein, 9 aa, synthetic construct
GGLGMDTAV

SEQ ID NO: 14494 - protein, 9 aa, synthetic construct
GGNGDDQLF

SEQ ID NO: 14495 - protein, 9 aa, synthetic construct
GGPGKDNLR

SEQ ID NO: 14496 - protein, 9 aa, synthetic construct
GGEGDDKIF

SEQ ID NO: 14497 - protein, 9 aa, synthetic construct
GGAGVDSIT

SEQ ID NO: 14498 - protein, 9 aa, synthetic construct
GGPGKDMLY

SEQ ID NO: 14499 - protein, 9 aa, synthetic construct
GGYGADVLI

SEQ ID NO: 14500 - protein, 9 aa, synthetic construct
GGPGADDFV

SEQ ID NO: 14501 - protein, 9 aa, synthetic construct
GGAGADVFF

SEQ ID NO: 14502 - protein, 9 aa, synthetic construct
GGVGVDVLT

SEQ ID NO: 14503 - protein, 9 aa, synthetic construct
GGSGSDRIA

SEQ ID NO: 14504 - protein, 9 aa, synthetic construct
GGFGGDPYG

SEQ ID NO: 14505 - protein, 9 aa, synthetic construct
GGAGVDRIS

SEQ ID NO: 14506 - protein, 9 aa, synthetic construct
GGDGIDDLM

SEQ ID NO: 14507 - protein, 9 aa, synthetic construct
GGMGDDRLY

SEQ ID NO: 14508 - protein, 9 aa, synthetic construct
GGGGYDRIK

SEQ ID NO: 14509 - protein, 9 aa, synthetic construct
GGSGSDRFI

SEQ ID NO: 14510 - protein, 9 aa, synthetic construct
GGDGADEFI

SEQ ID NO: 14511 - protein, 9 aa, synthetic construct
GGSGSDELL

SEQ ID NO: 14512 - protein, 9 aa, synthetic construct
GGEGRDLLR

SEQ ID NO: 14513 - protein, 9 aa, synthetic construct
GGGGKDKLA

SEQ ID NO: 14514 - protein, 9 aa, synthetic construct
GGEGRDLLT

SEQ ID NO: 14515 - protein, 9 aa, synthetic construct
GGSGNDVAL

SEQ ID NO: 14516 - protein, 9 aa, synthetic construct
GGVGVDTMI

SEQ ID NO: 14517 - protein, 9 aa, synthetic construct
GGGGTDTFI

SEQ ID NO: 14518 - protein, 9 aa, synthetic construct
GGGGDDVIA

SEQ ID NO: 14519 - protein, 9 aa, synthetic construct
GGLGPDRMI

SEQ ID NO: 14520 - protein, 9 aa, synthetic construct
GGNGNDLAE

SEQ ID NO: 14521 - protein, 9 aa, synthetic construct
GGMGGDTLT

SEQ ID NO: 14522 - protein, 9 aa, synthetic construct
GGPGADAFI

SEQ ID NO: 14523 - protein, 9 aa, synthetic construct
GGPGADAFM

SEQ ID NO: 14524 - protein, 9 aa, synthetic construct
GGPGADAIH

SEQ ID NO: 14525 - protein, 9 aa, synthetic construct
GGLGLDYLN

SEQ ID NO: 14526 - protein, 9 aa, synthetic construct
GGDGADDMS

SEQ ID NO: 14527 - protein, 9 aa, synthetic construct
GGGGDDVIE

SEQ ID NO: 14528 - protein, 9 aa, synthetic construct
GGDGADDMA

SEQ ID NO: 14529 - protein, 9 aa, synthetic construct
GGVGYDQLA

SEQ ID NO: 14530 - protein, 9 aa, synthetic construct
GGPGLDILD

SEQ ID NO: 14531 - protein, 9 aa, synthetic construct
GGPGLDIAS

SEQ ID NO: 14532 - protein, 9 aa, synthetic construct
GGMGDDRYV

SEQ ID NO: 14533 - protein, 9 aa, synthetic construct
GGPGGDRLA

SEQ ID NO: 14534 - protein, 9 aa, synthetic construct
GGGGVDVLV

SEQ ID NO: 14535 - protein, 9 aa, synthetic construct
GGLGNDDLY

SEQ ID NO: 14536 - protein, 9 aa, synthetic construct
GGGGKDLLI

SEQ ID NO: 14537 - protein, 9 aa, synthetic construct
GGAGADRIL

SEQ ID NO: 14538 - protein, 9 aa, synthetic construct
GGGGNDRMI

SEQ ID NO: 14539 - protein, 9 aa, synthetic construct
GGLGNDIFV

SEQ ID NO: 14540 - protein, 9 aa, synthetic construct
GGDGEDVFV

SEQ ID NO: 14541 - protein, 9 aa, synthetic construct
GGDGHDSIS

SEQ ID NO: 14542 - protein, 9 aa, synthetic construct
GGAGLDSLY

SEQ ID NO: 14543 - protein, 9 aa, synthetic construct
GGAGADRIQ

SEQ ID NO: 14544 - protein, 9 aa, synthetic construct
GGDGHDRLN

SEQ ID NO: 14545 - protein, 9 aa, synthetic construct
GGNGNDNLT

SEQ ID NO: 14546 - protein, 9 aa, synthetic construct
GGLGNDIFH

SEQ ID NO: 14547 - protein, 9 aa, synthetic construct
GGKGDDTYT

SEQ ID NO: 14548 - protein, 9 aa, synthetic construct
GGWGNDQLY

SEQ ID NO: 14549 - protein, 9 aa, synthetic construct
GGGGDDSFY

SEQ ID NO: 14550 - protein, 9 aa, synthetic construct
GGGGHDVLL

SEQ ID NO: 14551 - protein, 9 aa, synthetic construct
GGLGNDIIF

SEQ ID NO: 14552 - protein, 9 aa, synthetic construct
GGAGWDVVD

SEQ ID NO: 14553 - protein, 9 aa, synthetic construct
GGDGNDVFK

SEQ ID NO: 14554 - protein, 9 aa, synthetic construct
GGGGDDSIL

SEQ ID NO: 14555 - protein, 9 aa, synthetic construct
GGGGVDSFD

SEQ ID NO: 14556 - protein, 9 aa, synthetic construct
GGWGNDRVD

SEQ ID NO: 14557 - protein, 9 aa, synthetic construct
GGAGADQIV

SEQ ID NO: 14558 - protein, 9 aa, synthetic construct
GGEGADKLW

SEQ ID NO: 14559 - protein, 9 aa, synthetic construct
GGPGDDRLS

SEQ ID NO: 14560 - protein, 9 aa, synthetic construct
GGEGEDKLY

SEQ ID NO: 14561 - protein, 9 aa, synthetic construct
GGNGNDNLN

SEQ ID NO: 14562 - protein, 9 aa, synthetic construct
GGDGHDSLD

SEQ ID NO: 14563 - protein, 9 aa, synthetic construct
GGPGDDRLE

SEQ ID NO: 14564 - protein, 9 aa, synthetic construct
GGEGKDVLV

SEQ ID NO: 14565 - protein, 9 aa, synthetic construct
GGDGHDSVW

SEQ ID NO: 14566 - protein, 9 aa, synthetic construct
GGGGVDRLV

SEQ ID NO: 14567 - protein, 9 aa, synthetic construct
GGGGDDSIV

SEQ ID NO: 14568 - protein, 9 aa, synthetic construct
GGAGYDRLY

SEQ ID NO: 14569 - protein, 9 aa, synthetic construct
GGDGADVLH

SEQ ID NO: 14570 - protein, 9 aa, synthetic construct
GGNGNDNLY

SEQ ID NO: 14571 - protein, 9 aa, synthetic construct
GGGGVDIAS

SEQ ID NO: 14572 - protein, 9 aa, synthetic construct
GGDGFDYLN

SEQ ID NO: 14573 - protein, 9 aa, synthetic construct
GGLGPDVLV

SEQ ID NO: 14574 - protein, 9 aa, synthetic construct
GGPGDDDMT

SEQ ID NO: 14575 - protein, 9 aa, synthetic construct
GGDGDDLMT

SEQ ID NO: 14576 - protein, 9 aa, synthetic construct
GGSGSDHLL

SEQ ID NO: 14577 - protein, 9 aa, synthetic construct
GGEGRDRID

SEQ ID NO: 14578 - protein, 9 aa, synthetic construct
GGEGQDRLT

SEQ ID NO: 14579 - protein, 9 aa, synthetic construct
GGSGNDYLT

SEQ ID NO: 14580 - protein, 9 aa, synthetic construct
GGDGHDTLE

SEQ ID NO: 14581 - protein, 9 aa, synthetic construct
GGAGKDRFE

SEQ ID NO: 14582 - protein, 9 aa, synthetic construct
GGDGVDVLD

SEQ ID NO: 14583 - protein, 9 aa, synthetic construct
GGAGADRIY

SEQ ID NO: 14584 - protein, 9 aa, synthetic construct
GGAGYDTAG

SEQ ID NO: 14585 - protein, 9 aa, synthetic construct
GGPGDDTLF

SEQ ID NO: 14586 - protein, 9 aa, synthetic construct
GGGGSDALY

SEQ ID NO: 14587 - protein, 9 aa, synthetic construct
GGNGNDMIG

SEQ ID NO: 14588 - protein, 9 aa, synthetic construct
GGAGKDRLT

SEQ ID NO: 14589 - protein, 9 aa, synthetic construct
GGWGNDLLS

SEQ ID NO: 14590 - protein, 9 aa, synthetic construct
GGGGVDSLT

SEQ ID NO: 14591 - protein, 9 aa, synthetic construct
GGEGRDSID

SEQ ID NO: 14592 - protein, 9 aa, synthetic construct
GGAGYDSLS

SEQ ID NO: 14593 - protein, 9 aa, synthetic construct
GGNGNDLVV

SEQ ID NO: 14594 - protein, 9 aa, synthetic construct
GGMGDDVYL

SEQ ID NO: 14595 - protein, 9 aa, synthetic construct
GGLGNDHME

SEQ ID NO: 14596 - protein, 9 aa, synthetic construct
GGSGNDWMF

SEQ ID NO: 14597 - protein, 9 aa, synthetic construct
GGWGSDRVR

SEQ ID NO: 14598 - protein, 9 aa, synthetic construct
GGNGNDNMR

SEQ ID NO: 14599 - protein, 9 aa, synthetic construct
GGAGYDRVE

SEQ ID NO: 14600 - protein, 9 aa, synthetic construct
GGSGSDIYI

SEQ ID NO: 14601 - protein, 9 aa, synthetic construct
GGDGHDTIN

SEQ ID NO: 14602 - protein, 9 aa, synthetic construct
GGSGSDIMR

SEQ ID NO: 14603 - protein, 9 aa, synthetic construct
GGGGVDRLL

SEQ ID NO: 14604 - protein, 9 aa, synthetic construct
GGEGDDRIS

SEQ ID NO: 14605 - protein, 9 aa, synthetic construct
GGFGNDILL

SEQ ID NO: 14606 - protein, 9 aa, synthetic construct
GGPGDDILR

SEQ ID NO: 14607 - protein, 9 aa, synthetic construct
GGEGRDRLT

SEQ ID NO: 14608 - protein, 9 aa, synthetic construct
GGEGADKMW

SEQ ID NO: 14609 - protein, 9 aa, synthetic construct
GGWGNDYLD

SEQ ID NO: 14610 - protein, 9 aa, synthetic construct
GGDGEDILN

SEQ ID NO: 14611 - protein, 9 aa, synthetic construct
GGGGVDKLY

SEQ ID NO: 14612 - protein, 9 aa, synthetic construct
GGAGKDRLE

SEQ ID NO: 14613 - protein, 9 aa, synthetic construct
GGDGEDILI

SEQ ID NO: 14614 - protein, 9 aa, synthetic construct
GGEGADLAD

SEQ ID NO: 14615 - protein, 9 aa, synthetic construct
GGPGDDLLM

SEQ ID NO: 14616 - protein, 9 aa, synthetic construct
GGLGNDIYT

SEQ ID NO: 14617 - protein, 9 aa, synthetic construct
GGGGGDVMY

SEQ ID NO: 14618 - protein, 9 aa, synthetic construct
GGLGNDIYR

SEQ ID NO: 14619 - protein, 9 aa, synthetic construct
GGMGDDTYF

SEQ ID NO: 14620 - protein, 9 aa, synthetic construct
GGEGDDSIE

SEQ ID NO: 14621 - protein, 9 aa, synthetic construct
GGPGDDILN

SEQ ID NO: 14622 - protein, 9 aa, synthetic construct
GGPGDDLLD

SEQ ID NO: 14623 - protein, 9 aa, synthetic construct
GGNGNDMVT

SEQ ID NO: 14624 - protein, 9 aa, synthetic construct
GGWGRDSLS

SEQ ID NO: 14625 - protein, 9 aa, synthetic construct
GGLGNDIYF

SEQ ID NO: 14626 - protein, 9 aa, synthetic construct
GGDGHDSLS

SEQ ID NO: 14627 - protein, 9 aa, synthetic construct
GGWGRDKVY

SEQ ID NO: 14628 - protein, 9 aa, synthetic construct
GGNGNDNIV

SEQ ID NO: 14629 - protein, 9 aa, synthetic construct
GGLGNDIMF

SEQ ID NO: 14630 - protein, 9 aa, synthetic construct
GGLGNDIVV

SEQ ID NO: 14631 - protein, 9 aa, synthetic construct
GGEGADVIN

SEQ ID NO: 14632 - protein, 9 aa, synthetic construct
GGAGKDRLA

SEQ ID NO: 14633 - protein, 9 aa, synthetic construct
GGDGHDSLV

SEQ ID NO: 14634 - protein, 9 aa, synthetic construct
GGAGADQMA

SEQ ID NO: 14635 - protein, 9 aa, synthetic construct
GGAGLDSIE

SEQ ID NO: 14636 - protein, 9 aa, synthetic construct
GGGGDDSLW

SEQ ID NO: 14637 - protein, 9 aa, synthetic construct
GGNGDDRIF

SEQ ID NO: 14638 - protein, 9 aa, synthetic construct
GGAGYDQVD

SEQ ID NO: 14639 - protein, 9 aa, synthetic construct
GGWGNDTLI

SEQ ID NO: 14640 - protein, 9 aa, synthetic construct
GGPGDDRIA

SEQ ID NO: 14641 - protein, 9 aa, synthetic construct
GGDGEDILT

SEQ ID NO: 14642 - protein, 9 aa, synthetic construct
GGAGADQIW

SEQ ID NO: 14643 - protein, 9 aa, synthetic construct
GGDGADVIT

SEQ ID NO: 14644 - protein, 9 aa, synthetic construct
GGPGDDQLT

SEQ ID NO: 14645 - protein, 9 aa, synthetic construct
GGSGNDYFD

SEQ ID NO: 14646 - protein, 9 aa, synthetic construct
GGDGNDYFY

SEQ ID NO: 14647 - protein, 9 aa, synthetic construct
GGDGADVIV

SEQ ID NO: 14648 - protein, 9 aa, synthetic construct
GGPGDDIIL

SEQ ID NO: 14649 - protein, 9 aa, synthetic construct
GGNGDDRIS

SEQ ID NO: 14650 - protein, 9 aa, synthetic construct
GGPGDDIIS

SEQ ID NO: 14651 - protein, 9 aa, synthetic construct
GGAGADRFQ

SEQ ID NO: 14652 - protein, 9 aa, synthetic construct
GGAGYDELY

SEQ ID NO: 14653 - protein, 9 aa, synthetic construct
GGWGNDTIY

SEQ ID NO: 14654 - protein, 9 aa, synthetic construct
GGSGNDYIH

SEQ ID NO: 14655 - protein, 9 aa, synthetic construct
GGGGDDSYI

SEQ ID NO: 14656 - protein, 9 aa, synthetic construct
GGGGDDSLH

SEQ ID NO: 14657 - protein, 9 aa, synthetic construct
GGWGNDTLY

SEQ ID NO: 14658 - protein, 9 aa, synthetic construct
GGWGNDTVF

SEQ ID NO: 14659 - protein, 9 aa, synthetic construct
GGSGSDILF

SEQ ID NO: 14660 - protein, 9 aa, synthetic construct
GGEGDDSIG

SEQ ID NO: 14661 - protein, 9 aa, synthetic construct
GGAGADRAF

SEQ ID NO: 14662 - protein, 9 aa, synthetic construct
GGWGNDVIY

SEQ ID NO: 14663 - protein, 9 aa, synthetic construct
GGLGNDKIS

SEQ ID NO: 14664 - protein, 9 aa, synthetic construct
GGWGNDVLD

SEQ ID NO: 14665 - protein, 9 aa, synthetic construct
GGAGYDILN

SEQ ID NO: 14666 - protein, 9 aa, synthetic construct
GGAGADRAA

SEQ ID NO: 14667 - protein, 9 aa, synthetic construct
GGAGADQYA

SEQ ID NO: 14668 - protein, 9 aa, synthetic construct
GGGGVDKFF

SEQ ID NO: 14669 - protein, 9 aa, synthetic construct
GGDGVDWLD

SEQ ID NO: 14670 - protein, 9 aa, synthetic construct
GGDGADVLM

SEQ ID NO: 14671 - protein, 9 aa, synthetic construct
GGAGADRMH

SEQ ID NO: 14672 - protein, 9 aa, synthetic construct
GGDGWDRLL

SEQ ID NO: 14673 - protein, 9 aa, synthetic construct
GGPGEDWIF

SEQ ID NO: 14674 - protein, 9 aa, synthetic construct
GGGGDDTLW

SEQ ID NO: 14675 - protein, 9 aa, synthetic construct
GGLGNDELD

SEQ ID NO: 14676 - protein, 9 aa, synthetic construct
GGYGADKLT

SEQ ID NO: 14677 - protein, 9 aa, synthetic construct
GGEGRDTAS

SEQ ID NO: 14678 - protein, 9 aa, synthetic construct
GGAGADSMK

SEQ ID NO: 14679 - protein, 9 aa, synthetic construct
GGSGSDLLL

SEQ ID NO: 14680 - protein, 9 aa, synthetic construct
GGEGEDRLR

SEQ ID NO: 14681 - protein, 9 aa, synthetic construct
GGAGVDVLI

SEQ ID NO: 14682 - protein, 9 aa, synthetic construct
GGYGADKFI

SEQ ID NO: 14683 - protein, 9 aa, synthetic construct
GGGGTDVIV

SEQ ID NO: 14684 - protein, 9 aa, synthetic construct
GGLGNDELR

SEQ ID NO: 14685 - protein, 9 aa, synthetic construct
GGGGTDVLD

SEQ ID NO: 14686 - protein, 9 aa, synthetic construct
GGPGADVFV

SEQ ID NO: 14687 - protein, 9 aa, synthetic construct
GGDGYDDLY

SEQ ID NO: 14688 - protein, 9 aa, synthetic construct
GGMGDDTIY

SEQ ID NO: 14689 - protein, 9 aa, synthetic construct
GGLGPDVFR

SEQ ID NO: 14690 - protein, 9 aa, synthetic construct
GGGGDDQVF

SEQ ID NO: 14691 - protein, 9 aa, synthetic construct
GGDGHDTVF

SEQ ID NO: 14692 - protein, 9 aa, synthetic construct
GGAGADNID

SEQ ID NO: 14693 - protein, 9 aa, synthetic construct
GGSGSDLLA

SEQ ID NO: 14694 - protein, 9 aa, synthetic construct
GGSGNDVVL

SEQ ID NO: 14695 - protein, 9 aa, synthetic construct
GGAGVDWIY

SEQ ID NO: 14696 - protein, 9 aa, synthetic construct
GGAGLDRVI

SEQ ID NO: 14697 - protein, 9 aa, synthetic construct
GGLGNDLLM

SEQ ID NO: 14698 - protein, 9 aa, synthetic construct
GGAGVDWLV

SEQ ID NO: 14699 - protein, 9 aa, synthetic construct
GGGGVDTLV

SEQ ID NO: 14700 - protein, 9 aa, synthetic construct
GGAGADNIT

SEQ ID NO: 14701 - protein, 9 aa, synthetic construct
GGGGDDTLM

SEQ ID NO: 14702 - protein, 9 aa, synthetic construct
GGGGDDRFI

SEQ ID NO: 14703 - protein, 9 aa, synthetic construct
GGPGADVLT

SEQ ID NO: 14704 - protein, 9 aa, synthetic construct
GGAGADMLS

SEQ ID NO: 14705 - protein, 9 aa, synthetic construct
GGEGEDRLS

SEQ ID NO: 14706 - protein, 9 aa, synthetic construct
GGWGFDLVN

SEQ ID NO: 14707 - protein, 9 aa, synthetic construct
GGDGEDEIL

SEQ ID NO: 14708 - protein, 9 aa, synthetic construct
GGPGADTFL

SEQ ID NO: 14709 - protein, 9 aa, synthetic construct
GGAGLDRLV

SEQ ID NO: 14710 - protein, 9 aa, synthetic construct
GGDGHDVIT

SEQ ID NO: 14711 - protein, 9 aa, synthetic construct
GGAGLDTIS

SEQ ID NO: 14712 - protein, 9 aa, synthetic construct
GGPGGDLLE

SEQ ID NO: 14713 - protein, 9 aa, synthetic construct
GGPGGDLFH

SEQ ID NO: 14714 - protein, 9 aa, synthetic construct
GGEGDDRIF

SEQ ID NO: 14715 - protein, 9 aa, synthetic construct
GGEGNDYLV

SEQ ID NO: 14716 - protein, 9 aa, synthetic construct
GGGGKDRID

SEQ ID NO: 14717 - protein, 9 aa, synthetic construct
GGAGADMLL

SEQ ID NO: 14718 - protein, 9 aa, synthetic construct
GGLGNDDVR

SEQ ID NO: 14719 - protein, 9 aa, synthetic construct
GGAGVDTVT

SEQ ID NO: 14720 - protein, 9 aa, synthetic construct
GGKGDDVLD

SEQ ID NO: 14721 - protein, 9 aa, synthetic construct
GGLGVDVLD

SEQ ID NO: 14722 - protein, 9 aa, synthetic construct
GGPGADTIH

SEQ ID NO: 14723 - protein, 9 aa, synthetic construct
GGPGADTMT

SEQ ID NO: 14724 - protein, 9 aa, synthetic construct
GGLGNDLVD

SEQ ID NO: 14725 - protein, 9 aa, synthetic construct
GGLGVDVLT

SEQ ID NO: 14726 - protein, 9 aa, synthetic construct
GGAGADMLM

SEQ ID NO: 14727 - protein, 9 aa, synthetic construct
GGLGVDVLW

SEQ ID NO: 14728 - protein, 9 aa, synthetic construct
GGWGDDVLT

SEQ ID NO: 14729 - protein, 9 aa, synthetic construct
GGDGYDHIF

SEQ ID NO: 14730 - protein, 9 aa, synthetic construct
GGEGDDIVF

SEQ ID NO: 14731 - protein, 9 aa, synthetic construct
GGEGDDIVK

SEQ ID NO: 14732 - protein, 9 aa, synthetic construct
GGSGNDVMN

SEQ ID NO: 14733 - protein, 9 aa, synthetic construct
GGDGHDVAD

SEQ ID NO: 14734 - protein, 9 aa, synthetic construct
GGLGNDEIT

SEQ ID NO: 14735 - protein, 9 aa, synthetic construct
GGNGDDRLG

SEQ ID NO: 14736 - protein, 9 aa, synthetic construct
GGAGVDVID

SEQ ID NO: 14737 - protein, 9 aa, synthetic construct
GGGGDDTMF

SEQ ID NO: 14738 - protein, 9 aa, synthetic construct
GGEGEDRLD

SEQ ID NO: 14739 - protein, 9 aa, synthetic construct
GGLGNDFIN

SEQ ID NO: 14740 - protein, 9 aa, synthetic construct
GGGGVDTAI

SEQ ID NO: 14741 - protein, 9 aa, synthetic construct
GGEGADLIE

SEQ ID NO: 14742 - protein, 9 aa, synthetic construct
GGPGDDVLY

SEQ ID NO: 14743 - protein, 9 aa, synthetic construct
GGKGADVMI

SEQ ID NO: 14744 - protein, 9 aa, synthetic construct
GGDGWDTLQ

SEQ ID NO: 14745 - protein, 9 aa, synthetic construct
GGPGDDVLV

SEQ ID NO: 14746 - protein, 9 aa, synthetic construct
GGDGVDTVV

SEQ ID NO: 14747 - protein, 9 aa, synthetic construct
GGPGDDVLS

SEQ ID NO: 14748 - protein, 9 aa, synthetic construct
GGWGKDQFV

SEQ ID NO: 14749 - protein, 9 aa, synthetic construct
GGPGDDVLN

SEQ ID NO: 14750 - protein, 9 aa, synthetic construct
GGSGSDHAV

SEQ ID NO: 14751 - protein, 9 aa, synthetic construct
GGPGDDVLH

SEQ ID NO: 14752 - protein, 9 aa, synthetic construct
GGAGADNVS

SEQ ID NO: 14753 - protein, 9 aa, synthetic construct
GGAGLDTAR

SEQ ID NO: 14754 - protein, 9 aa, synthetic construct
GGPGDDVLE

SEQ ID NO: 14755 - protein, 9 aa, synthetic construct
GGPGDDALF

SEQ ID NO: 14756 - protein, 9 aa, synthetic construct
GGAGADQFL

SEQ ID NO: 14757 - protein, 9 aa, synthetic construct
GGAGYDTVG

SEQ ID NO: 14758 - protein, 9 aa, synthetic construct
GGPGDDVIS

SEQ ID NO: 14759 - protein, 9 aa, synthetic construct
GGDGHDTLI

SEQ ID NO: 14760 - protein, 9 aa, synthetic construct
GGNGDDRIW

SEQ ID NO: 14761 - protein, 9 aa, synthetic construct
GGPGDDVIF

SEQ ID NO: 14762 - protein, 9 aa, synthetic construct
GGLGNDGLR

SEQ ID NO: 14763 - protein, 9 aa, synthetic construct
GGNGNDQIF

SEQ ID NO: 14764 - protein, 9 aa, synthetic construct
GGDGWDRLW

SEQ ID NO: 14765 - protein, 9 aa, synthetic construct
GGAGYDTFL

SEQ ID NO: 14766 - protein, 9 aa, synthetic construct
GGWGSDVIY

SEQ ID NO: 14767 - protein, 9 aa, synthetic construct
GGAGWDSVN

SEQ ID NO: 14768 - protein, 9 aa, synthetic construct
GGGGDDTIH

SEQ ID NO: 14769 - protein, 9 aa, synthetic construct
GGLGNDLII

SEQ ID NO: 14770 - protein, 9 aa, synthetic construct
GGWGNDALH

SEQ ID NO: 14771 - protein, 9 aa, synthetic construct
GGAGWDTAL

SEQ ID NO: 14772 - protein, 9 aa, synthetic construct
GGNGNDQIL

SEQ ID NO: 14773 - protein, 9 aa, synthetic construct
GGPGADYLD

SEQ ID NO: 14774 - protein, 9 aa, synthetic construct
GGAGYDVLT

SEQ ID NO: 14775 - protein, 9 aa, synthetic construct
GGSGNDVYR

SEQ ID NO: 14776 - protein, 9 aa, synthetic construct
GGAGLDTFV

SEQ ID NO: 14777 - protein, 9 aa, synthetic construct
GGKGDDDLY

SEQ ID NO: 14778 - protein, 9 aa, synthetic construct
GGDGYDAIY

SEQ ID NO: 14779 - protein, 9 aa, synthetic construct
GGAGADSIR

SEQ ID NO: 14780 - protein, 9 aa, synthetic construct
GGAGVDYLH

SEQ ID NO: 14781 - protein, 9 aa, synthetic construct
GGAGYDVLI

SEQ ID NO: 14782 - protein, 9 aa, synthetic construct
GGGGDDRIG

SEQ ID NO: 14783 - protein, 9 aa, synthetic construct
GGLGNDFLH

SEQ ID NO: 14784 - protein, 9 aa, synthetic construct
GGKGADVLV

SEQ ID NO: 14785 - protein, 9 aa, synthetic construct
GGSGSDLFL

SEQ ID NO: 14786 - protein, 9 aa, synthetic construct
GGAGVDYLY

SEQ ID NO: 14787 - protein, 9 aa, synthetic construct
GGMGDDTLH

SEQ ID NO: 14788 - protein, 9 aa, synthetic construct
GGGGDDRIL

SEQ ID NO: 14789 - protein, 9 aa, synthetic construct
GGSGNDVYN

SEQ ID NO: 14790 - protein, 9 aa, synthetic construct
GGLGNDLLG

SEQ ID NO: 14791 - protein, 9 aa, synthetic construct
GGPGDDVVE

SEQ ID NO: 14792 - protein, 9 aa, synthetic construct
GGEGNDAIY

SEQ ID NO: 14793 - protein, 9 aa, synthetic construct
GGGGVDTLM

SEQ ID NO: 14794 - protein, 9 aa, synthetic construct
GGLGYDFID

SEQ ID NO: 14795 - protein, 9 aa, synthetic construct
GGSGNDWAS

SEQ ID NO: 14796 - protein, 9 aa, synthetic construct
GGFGHDQIG

SEQ ID NO: 14797 - protein, 9 aa, synthetic construct
GGWGHDRVN

SEQ ID NO: 14798 - protein, 9 aa, synthetic construct
GGSGNDYVE

SEQ ID NO: 14799 - protein, 9 aa, synthetic construct
GGWGHDTLL

SEQ ID NO: 14800 - protein, 9 aa, synthetic construct
GGGGGDVLK

SEQ ID NO: 14801 - protein, 9 aa, synthetic construct
GGEGNDWLF

SEQ ID NO: 14802 - protein, 9 aa, synthetic construct
GGDGHDALA

SEQ ID NO: 14803 - protein, 9 aa, synthetic construct
GGGGGDVLN

SEQ ID NO: 14804 - protein, 9 aa, synthetic construct
GGGGVDTLD

SEQ ID NO: 14805 - protein, 9 aa, synthetic construct
GGAGADNML

SEQ ID NO: 14806 - protein, 9 aa, synthetic construct
GGGGTDRLV

SEQ ID NO: 14807 - protein, 9 aa, synthetic construct
GGDGVDRLY

SEQ ID NO: 14808 - protein, 9 aa, synthetic construct
GGLGHDTLY

SEQ ID NO: 14809 - protein, 9 aa, synthetic construct
GGAGDDAIG

SEQ ID NO: 14810 - protein, 9 aa, synthetic construct
GGVGRDIFV

SEQ ID NO: 14811 - protein, 9 aa, synthetic construct
GGDGADLIF

SEQ ID NO: 14812 - protein, 9 aa, synthetic construct
GGGGLDLAD

SEQ ID NO: 14813 - protein, 9 aa, synthetic construct
GGAGDDAIE

SEQ ID NO: 14814 - protein, 9 aa, synthetic construct
GGAGTDVLL

SEQ ID NO: 14815 - protein, 9 aa, synthetic construct
GGEGRDIVV

SEQ ID NO: 14816 - protein, 9 aa, synthetic construct
GGGGDDIIV

SEQ ID NO: 14817 - protein, 9 aa, synthetic construct
GGHGDDKID

SEQ ID NO: 14818 - protein, 9 aa, synthetic construct
GGDGADLII

SEQ ID NO: 14819 - protein, 9 aa, synthetic construct
GGAGTDVLD

SEQ ID NO: 14820 - protein, 9 aa, synthetic construct
GGAGTDVLA

SEQ ID NO: 14821 - protein, 9 aa, synthetic construct
GGDGADLIN

SEQ ID NO: 14822 - protein, 9 aa, synthetic construct
GGSGQDSLF

SEQ ID NO: 14823 - protein, 9 aa, synthetic construct
GGLGPDKLT

SEQ ID NO: 14824 - protein, 9 aa, synthetic construct
GGSGSDVLE

SEQ ID NO: 14825 - protein, 9 aa, synthetic construct
GGAGDDAIA

SEQ ID NO: 14826 - protein, 9 aa, synthetic construct
GGEGRDYLL

SEQ ID NO: 14827 - protein, 9 aa, synthetic construct
GGPGRDLIH

SEQ ID NO: 14828 - protein, 9 aa, synthetic construct
GGYGFDQLI

SEQ ID NO: 14829 - protein, 9 aa, synthetic construct
GGNGSDTFR

SEQ ID NO: 14830 - protein, 9 aa, synthetic construct
GGSGSDVIN

SEQ ID NO: 14831 - protein, 9 aa, synthetic construct
GGHGDDELF

SEQ ID NO: 14832 - protein, 9 aa, synthetic construct
GGPGRDKLV

SEQ ID NO: 14833 - protein, 9 aa, synthetic construct
GGSGNDSVE

SEQ ID NO: 14834 - protein, 9 aa, synthetic construct
GGMGLDLIF

SEQ ID NO: 14835 - protein, 9 aa, synthetic construct
GGDGADLID

SEQ ID NO: 14836 - protein, 9 aa, synthetic construct
GGEGADILK

SEQ ID NO: 14837 - protein, 9 aa, synthetic construct
GGEGDDRFF

SEQ ID NO: 14838 - protein, 9 aa, synthetic construct
GGMGKDYLS

SEQ ID NO: 14839 - protein, 9 aa, synthetic construct
GGDGADLIA

SEQ ID NO: 14840 - protein, 9 aa, synthetic construct
GGYGEDVLK

SEQ ID NO: 14841 - protein, 9 aa, synthetic construct
GGDGADLIR

SEQ ID NO: 14842 - protein, 9 aa, synthetic construct
GGLGIDTAS

SEQ ID NO: 14843 - protein, 9 aa, synthetic construct
GGPGRDRAS

SEQ ID NO: 14844 - protein, 9 aa, synthetic construct
GGNGDDSVL

SEQ ID NO: 14845 - protein, 9 aa, synthetic construct
GGNGSDRLN

SEQ ID NO: 14846 - protein, 9 aa, synthetic construct
GGSGNDSMA

SEQ ID NO: 14847 - protein, 9 aa, synthetic construct
GGSGRDVLV

SEQ ID NO: 14848 - protein, 9 aa, synthetic construct
GGEGADILH

SEQ ID NO: 14849 - protein, 9 aa, synthetic construct
GGNGNDRMS

SEQ ID NO: 14850 - protein, 9 aa, synthetic construct
GGKGDDIFT

SEQ ID NO: 14851 - protein, 9 aa, synthetic construct
GGDGNDWID

SEQ ID NO: 14852 - protein, 9 aa, synthetic construct
GGDGADLLG

SEQ ID NO: 14853 - protein, 9 aa, synthetic construct
GGPGRDTLA

SEQ ID NO: 14854 - protein, 9 aa, synthetic construct
GGNGNDHLD

SEQ ID NO: 14855 - protein, 9 aa, synthetic construct
GGLGIDSLF

SEQ ID NO: 14856 - protein, 9 aa, synthetic construct
GGYGGDTIT

SEQ ID NO: 14857 - protein, 9 aa, synthetic construct
GGYGGDTIS

SEQ ID NO: 14858 - protein, 9 aa, synthetic construct
GGGGSDIIA

SEQ ID NO: 14859 - protein, 9 aa, synthetic construct
GGGGDDIIH

SEQ ID NO: 14860 - protein, 9 aa, synthetic construct
GGFGNDLLI

SEQ ID NO: 14861 - protein, 9 aa, synthetic construct
GGVGQDVLS

SEQ ID NO: 14862 - protein, 9 aa, synthetic construct
GGAGDDAIW

SEQ ID NO: 14863 - protein, 9 aa, synthetic construct
GGPGRDSLY

SEQ ID NO: 14864 - protein, 9 aa, synthetic construct
GGSGNDSMD

SEQ ID NO: 14865 - protein, 9 aa, synthetic construct
GGAGTDVFR

SEQ ID NO: 14866 - protein, 9 aa, synthetic construct
GGAGLDTVA

SEQ ID NO: 14867 - protein, 9 aa, synthetic construct
GGGGDDIIR

SEQ ID NO: 14868 - protein, 9 aa, synthetic construct
GGPGRDRLL

SEQ ID NO: 14869 - protein, 9 aa, synthetic construct
GGGGTDFLY

SEQ ID NO: 14870 - protein, 9 aa, synthetic construct
GGPGRDRLI

SEQ ID NO: 14871 - protein, 9 aa, synthetic construct
GGNGSDSLN

SEQ ID NO: 14872 - protein, 9 aa, synthetic construct
GGSGQDSLR

SEQ ID NO: 14873 - protein, 9 aa, synthetic construct
GGSGNDSMN

SEQ ID NO: 14874 - protein, 9 aa, synthetic construct
GGNGSDSLS

SEQ ID NO: 14875 - protein, 9 aa, synthetic construct
GGEGNDVMT

SEQ ID NO: 14876 - protein, 9 aa, synthetic construct
GGGGSDIFS

SEQ ID NO: 14877 - protein, 9 aa, synthetic construct
GGSGQDSIT

SEQ ID NO: 14878 - protein, 9 aa, synthetic construct
GGDGADKLT

SEQ ID NO: 14879 - protein, 9 aa, synthetic construct
GGEGRDKIV

SEQ ID NO: 14880 - protein, 9 aa, synthetic construct
GGGGDDYIG

SEQ ID NO: 14881 - protein, 9 aa, synthetic construct
GGEGDDHLS

SEQ ID NO: 14882 - protein, 9 aa, synthetic construct
GGAGADIVS

SEQ ID NO: 14883 - protein, 9 aa, synthetic construct
GGEGRDKLI

SEQ ID NO: 14884 - protein, 9 aa, synthetic construct
GGKGADSLT

SEQ ID NO: 14885 - protein, 9 aa, synthetic construct
GGAGADIVY

SEQ ID NO: 14886 - protein, 9 aa, synthetic construct
GGAGADYML

SEQ ID NO: 14887 - protein, 9 aa, synthetic construct
GGDGGDALF

SEQ ID NO: 14888 - protein, 9 aa, synthetic construct
GGMGADALS

SEQ ID NO: 14889 - protein, 9 aa, synthetic construct
GGDGADWLV

SEQ ID NO: 14890 - protein, 9 aa, synthetic construct
GGNGSDTYV

SEQ ID NO: 14891 - protein, 9 aa, synthetic construct
GGDGADKLV

SEQ ID NO: 14892 - protein, 9 aa, synthetic construct
GGLGIDYLD

SEQ ID NO: 14893 - protein, 9 aa, synthetic construct
GGYGDDYLN

SEQ ID NO: 14894 - protein, 9 aa, synthetic construct
GGGGSDIFN

SEQ ID NO: 14895 - protein, 9 aa, synthetic construct
GGSGNDTAD

SEQ ID NO: 14896 - protein, 9 aa, synthetic construct
GGSGQDRLS

SEQ ID NO: 14897 - protein, 9 aa, synthetic construct
GGNGSDVID

SEQ ID NO: 14898 - protein, 9 aa, synthetic construct
GGNGNDIIE

SEQ ID NO: 14899 - protein, 9 aa, synthetic construct
GGGGTDILT

SEQ ID NO: 14900 - protein, 9 aa, synthetic construct
GGVGRDVLN

SEQ ID NO: 14901 - protein, 9 aa, synthetic construct
GGNGNDIIL

SEQ ID NO: 14902 - protein, 9 aa, synthetic construct
GGDGIDSLF

SEQ ID NO: 14903 - protein, 9 aa, synthetic construct
GGLGKDIFV

SEQ ID NO: 14904 - protein, 9 aa, synthetic construct
GGLGKDILI

SEQ ID NO: 14905 - protein, 9 aa, synthetic construct
GGAGVDDLA

SEQ ID NO: 14906 - protein, 9 aa, synthetic construct
GGDGIDSLD

SEQ ID NO: 14907 - protein, 9 aa, synthetic construct
GGNGNDIIQ

SEQ ID NO: 14908 - protein, 9 aa, synthetic construct
GGVGRDVLV

SEQ ID NO: 14909 - protein, 9 aa, synthetic construct
GGSGQDRME

SEQ ID NO: 14910 - protein, 9 aa, synthetic construct
GGDGIDTAN

SEQ ID NO: 14911 - protein, 9 aa, synthetic construct
GGEGRDWIA

SEQ ID NO: 14912 - protein, 9 aa, synthetic construct
GGAGKDKID

SEQ ID NO: 14913 - protein, 9 aa, synthetic construct
GGGGRDTLG

SEQ ID NO: 14914 - protein, 9 aa, synthetic construct
GGNGDDRMV

SEQ ID NO: 14915 - protein, 9 aa, synthetic construct
GGVGRDRLT

SEQ ID NO: 14916 - protein, 9 aa, synthetic construct
GGEGDDVMD

SEQ ID NO: 14917 - protein, 9 aa, synthetic construct
GGDGGDALI

SEQ ID NO: 14918 - protein, 9 aa, synthetic construct
GGVGRDSLF

SEQ ID NO: 14919 - protein, 9 aa, synthetic construct
GGAGTDWLI

SEQ ID NO: 14920 - protein, 9 aa, synthetic construct
GGDGADLFR

SEQ ID NO: 14921 - protein, 9 aa, synthetic construct
GGSGNDSVF

SEQ ID NO: 14922 - protein, 9 aa, synthetic construct
GGLGIDTLR

SEQ ID NO: 14923 - protein, 9 aa, synthetic construct
GGLGIDTLS

SEQ ID NO: 14924 - protein, 9 aa, synthetic construct
GGDGDDMAS

SEQ ID NO: 14925 - protein, 9 aa, synthetic construct
GGDGADWVD

SEQ ID NO: 14926 - protein, 9 aa, synthetic construct
GGYGEDTIR

SEQ ID NO: 14927 - protein, 9 aa, synthetic construct
GGNGSDTLR

SEQ ID NO: 14928 - protein, 9 aa, synthetic construct
GGAGVDALA

SEQ ID NO: 14929 - protein, 9 aa, synthetic construct
GGDGGDDLD

SEQ ID NO: 14930 - protein, 9 aa, synthetic construct
GGGGHDILI

SEQ ID NO: 14931 - protein, 9 aa, synthetic construct
GGGGDDIVN

SEQ ID NO: 14932 - protein, 9 aa, synthetic construct
GGHGADTLY

SEQ ID NO: 14933 - protein, 9 aa, synthetic construct
GGEGFDALY

SEQ ID NO: 14934 - protein, 9 aa, synthetic construct
GGDGNDYVY

SEQ ID NO: 14935 - protein, 9 aa, synthetic construct
GGPGQDVLD

SEQ ID NO: 14936 - protein, 9 aa, synthetic construct
GGSGNDSVY

SEQ ID NO: 14937 - protein, 9 aa, synthetic construct
GGYGEDRLV

SEQ ID NO: 14938 - protein, 9 aa, synthetic construct
GGVGRDTVN

SEQ ID NO: 14939 - protein, 9 aa, synthetic construct
GGNGSDTLV

SEQ ID NO: 14940 - protein, 9 aa, synthetic construct
GGEGDDHLQ

SEQ ID NO: 14941 - protein, 9 aa, synthetic construct
GGGGDDIYI

SEQ ID NO: 14942 - protein, 9 aa, synthetic construct
GGEGADLLT

SEQ ID NO: 14943 - protein, 9 aa, synthetic construct
GGGGKDFLI

SEQ ID NO: 14944 - protein, 9 aa, synthetic construct
GGAGDDALK

SEQ ID NO: 14945 - protein, 9 aa, synthetic construct
GGSGNDTVL

SEQ ID NO: 14946 - protein, 9 aa, synthetic construct
GGGGDDYLV

SEQ ID NO: 14947 - protein, 9 aa, synthetic construct
GGDGEDRLA

SEQ ID NO: 14948 - protein, 9 aa, synthetic construct
GGDGDDWVA

SEQ ID NO: 14949 - protein, 9 aa, synthetic construct
GGAGDDDIN

SEQ ID NO: 14950 - protein, 9 aa, synthetic construct
GGEGRDILY

SEQ ID NO: 14951 - protein, 9 aa, synthetic construct
GGNGSDIIY

SEQ ID NO: 14952 - protein, 9 aa, synthetic construct
GGNGNDGLI

SEQ ID NO: 14953 - protein, 9 aa, synthetic construct
GGYGKDILI

SEQ ID NO: 14954 - protein, 9 aa, synthetic construct
GGDGADLLK

SEQ ID NO: 14955 - protein, 9 aa, synthetic construct
GGNGNDGLF

SEQ ID NO: 14956 - protein, 9 aa, synthetic construct
GGDGADTYI

SEQ ID NO: 14957 - protein, 9 aa, synthetic construct
GGAGDDDIR

SEQ ID NO: 14958 - protein, 9 aa, synthetic construct
GGVGNDVMN

SEQ ID NO: 14959 - protein, 9 aa, synthetic construct
GGGGSDWLV

SEQ ID NO: 14960 - protein, 9 aa, synthetic construct
GGPGSDTLR

SEQ ID NO: 14961 - protein, 9 aa, synthetic construct
GGAGDDDIF

SEQ ID NO: 14962 - protein, 9 aa, synthetic construct
GGEGDDHLA

SEQ ID NO: 14963 - protein, 9 aa, synthetic construct
GGNGSDILN

SEQ ID NO: 14964 - protein, 9 aa, synthetic construct
GGEGDDHLD

SEQ ID NO: 14965 - protein, 9 aa, synthetic construct
GGNGSDILQ

SEQ ID NO: 14966 - protein, 9 aa, synthetic construct
GGGGSDILL

SEQ ID NO: 14967 - protein, 9 aa, synthetic construct
GGAGKDTIV

SEQ ID NO: 14968 - protein, 9 aa, synthetic construct
GGYGIDTII

SEQ ID NO: 14969 - protein, 9 aa, synthetic construct
GGDGIDTVS

SEQ ID NO: 14970 - protein, 9 aa, synthetic construct
GGDGVDHIE

SEQ ID NO: 14971 - protein, 9 aa, synthetic construct
GGVGNDWLD

SEQ ID NO: 14972 - protein, 9 aa, synthetic construct
GGSGRDVLH

SEQ ID NO: 14973 - protein, 9 aa, synthetic construct
GGDGNDWIA

SEQ ID NO: 14974 - protein, 9 aa, synthetic construct
GGGGSDYVD

SEQ ID NO: 14975 - protein, 9 aa, synthetic construct
GGDGADTYQ

SEQ ID NO: 14976 - protein, 9 aa, synthetic construct
GGNGNDRVN

SEQ ID NO: 14977 - protein, 9 aa, synthetic construct
GGNGSDLFH

SEQ ID NO: 14978 - protein, 9 aa, synthetic construct
GGPGSDTLS

SEQ ID NO: 14979 - protein, 9 aa, synthetic construct
GGPGSDTLT

SEQ ID NO: 14980 - protein, 9 aa, synthetic construct
GGDGADMLQ

SEQ ID NO: 14981 - protein, 9 aa, synthetic construct
GGKGDDYLL

SEQ ID NO: 14982 - protein, 9 aa, synthetic construct
GGSGQDTVD

SEQ ID NO: 14983 - protein, 9 aa, synthetic construct
GGEGSDEFH

SEQ ID NO: 14984 - protein, 9 aa, synthetic construct
GGSGRDTYT

SEQ ID NO: 14985 - protein, 9 aa, synthetic construct
GGAGTDSLV

SEQ ID NO: 14986 - protein, 9 aa, synthetic construct
GGAGTDSLW

SEQ ID NO: 14987 - protein, 9 aa, synthetic construct
GGEGRDILR

SEQ ID NO: 14988 - protein, 9 aa, synthetic construct
GGGGHDIII

SEQ ID NO: 14989 - protein, 9 aa, synthetic construct
GGAGTDSMD

SEQ ID NO: 14990 - protein, 9 aa, synthetic construct
GGEGFDFVS

SEQ ID NO: 14991 - protein, 9 aa, synthetic construct
GGDGADNID

SEQ ID NO: 14992 - protein, 9 aa, synthetic construct
GGSGQDTLV

SEQ ID NO: 14993 - protein, 9 aa, synthetic construct
GGPGSDVYV

SEQ ID NO: 14994 - protein, 9 aa, synthetic construct
GGGGSDWLD

SEQ ID NO: 14995 - protein, 9 aa, synthetic construct
GGDGIDVLS

SEQ ID NO: 14996 - protein, 9 aa, synthetic construct
GGLGHDVLI

SEQ ID NO: 14997 - protein, 9 aa, synthetic construct
GGSGSDYLL

SEQ ID NO: 14998 - protein, 9 aa, synthetic construct
GGDGADNFR

SEQ ID NO: 14999 - protein, 9 aa, synthetic construct
GGDGADMLY

SEQ ID NO: 15000 - protein, 9 aa, synthetic construct
GGAGTDSYI

SEQ ID NO: 15001 - protein, 9 aa, synthetic construct
GGDGADMLW

SEQ ID NO: 15002 - protein, 9 aa, synthetic construct
GGNGNDGLA

SEQ ID NO: 15003 - protein, 9 aa, synthetic construct
GGPGSDTYL

SEQ ID NO: 15004 - protein, 9 aa, synthetic construct
GGDGHDKLF

SEQ ID NO: 15005 - protein, 9 aa, synthetic construct
GGVGNDVLW

SEQ ID NO: 15006 - protein, 9 aa, synthetic construct
GGDGADMLS

SEQ ID NO: 15007 - protein, 9 aa, synthetic construct
GGGGGDTLS

SEQ ID NO: 15008 - protein, 9 aa, synthetic construct
GGDGDDLME

SEQ ID NO: 15009 - protein, 9 aa, synthetic construct
GGLGHDVLV

SEQ ID NO: 15010 - protein, 9 aa, synthetic construct
GGPGSDTMT

SEQ ID NO: 15011 - protein, 9 aa, synthetic construct
GGVGNDVMG

SEQ ID NO: 15012 - protein, 9 aa, synthetic construct
GGPGSDMLD

SEQ ID NO: 15013 - protein, 9 aa, synthetic construct
GGGGSDIIY

SEQ ID NO: 15014 - protein, 9 aa, synthetic construct
GGAGTDTIQ

SEQ ID NO: 15015 - protein, 9 aa, synthetic construct
GGAGTDTVL

SEQ ID NO: 15016 - protein, 9 aa, synthetic construct
GGDGADLML

SEQ ID NO: 15017 - protein, 9 aa, synthetic construct
GGYGHDTLR

SEQ ID NO: 15018 - protein, 9 aa, synthetic construct
GGLGNDSYR

SEQ ID NO: 15019 - protein, 9 aa, synthetic construct
GGAGLDIAA

SEQ ID NO: 15020 - protein, 9 aa, synthetic construct
GGYGHDTFY

SEQ ID NO: 15021 - protein, 9 aa, synthetic construct
GGPGRDVMI

SEQ ID NO: 15022 - protein, 9 aa, synthetic construct
GGSGQDTID

SEQ ID NO: 15023 - protein, 9 aa, synthetic construct
GGAGTDTMT

SEQ ID NO: 15024 - protein, 9 aa, synthetic construct
GGAGTDTMV

SEQ ID NO: 15025 - protein, 9 aa, synthetic construct
GGDGADLLW

SEQ ID NO: 15026 - protein, 9 aa, synthetic construct
GGKGADSFY

SEQ ID NO: 15027 - protein, 9 aa, synthetic construct
GGDGIDTLR

SEQ ID NO: 15028 - protein, 9 aa, synthetic construct
GGGGSDIII

SEQ ID NO: 15029 - protein, 9 aa, synthetic construct
GGEGRDIVF

SEQ ID NO: 15030 - protein, 9 aa, synthetic construct
GGDGDDMIA

SEQ ID NO: 15031 - protein, 9 aa, synthetic construct
GGAGADIIS

SEQ ID NO: 15032 - protein, 9 aa, synthetic construct
GGAGTDTVN

SEQ ID NO: 15033 - protein, 9 aa, synthetic construct
GGSGQDTFV

SEQ ID NO: 15034 - protein, 9 aa, synthetic construct
GGEGSDALA

SEQ ID NO: 15035 - protein, 9 aa, synthetic construct
GGMGDDIYI

SEQ ID NO: 15036 - protein, 9 aa, synthetic construct
GGSGSDVMR

SEQ ID NO: 15037 - protein, 9 aa, synthetic construct
GGDGVDIAV

SEQ ID NO: 15038 - protein, 9 aa, synthetic construct
GGNGSDRLA

SEQ ID NO: 15039 - protein, 9 aa, synthetic construct
GGSGSDVLT

SEQ ID NO: 15040 - protein, 9 aa, synthetic construct
GGSGSDVLR

SEQ ID NO: 15041 - protein, 9 aa, synthetic construct
GGVGQDRLE

SEQ ID NO: 15042 - protein, 9 aa, synthetic construct
GGAGADILG

SEQ ID NO: 15043 - protein, 9 aa, synthetic construct
GGNGSDRLE

SEQ ID NO: 15044 - protein, 9 aa, synthetic construct
GGDGYDTLY

SEQ ID NO: 15045 - protein, 9 aa, synthetic construct
GGGGDDIIF

SEQ ID NO: 15046 - protein, 9 aa, synthetic construct
GGEGDDVVL

SEQ ID NO: 15047 - protein, 9 aa, synthetic construct
GGLGIDLLS

SEQ ID NO: 15048 - protein, 9 aa, synthetic construct
GGLGNDTAS

SEQ ID NO: 15049 - protein, 9 aa, synthetic construct
GGLGNDTAL

SEQ ID NO: 15050 - protein, 9 aa, synthetic construct
GGAGTDTIS

SEQ ID NO: 15051 - protein, 9 aa, synthetic construct
GGAGTDTIT

SEQ ID NO: 15052 - protein, 9 aa, synthetic construct
GGNGSDLIY

SEQ ID NO: 15053 - protein, 9 aa, synthetic construct
GGGGDDIFT

SEQ ID NO: 15054 - protein, 9 aa, synthetic construct
GGNGSDLLE

SEQ ID NO: 15055 - protein, 9 aa, synthetic construct
GGKGDDRLD

SEQ ID NO: 15056 - protein, 9 aa, synthetic construct
GGEGSDAVR

SEQ ID NO: 15057 - protein, 9 aa, synthetic construct
GGDGDDMIE

SEQ ID NO: 15058 - protein, 9 aa, synthetic construct
GGAGKDIMN

SEQ ID NO: 15059 - protein, 9 aa, synthetic construct
GGVGNDYLR

SEQ ID NO: 15060 - protein, 9 aa, synthetic construct
GGVGNDYLY

SEQ ID NO: 15061 - protein, 9 aa, synthetic construct
GGEGADILD

SEQ ID NO: 15062 - protein, 9 aa, synthetic construct
GGEGDDYII

SEQ ID NO: 15063 - protein, 9 aa, synthetic construct
GGNGSDLLY

SEQ ID NO: 15064 - protein, 9 aa, synthetic construct
GGLGNDTAI

SEQ ID NO: 15065 - protein, 9 aa, synthetic construct
GGYGHDTLV

SEQ ID NO: 15066 - protein, 9 aa, synthetic construct
GGAGTDTLM

SEQ ID NO: 15067 - protein, 9 aa, synthetic construct
GGYGHDVLT

SEQ ID NO: 15068 - protein, 9 aa, synthetic construct
GGHGDDLLS

SEQ ID NO: 15069 - protein, 9 aa, synthetic construct
GGVGPDLIQ

SEQ ID NO: 15070 - protein, 9 aa, synthetic construct
GGDGADYIE

SEQ ID NO: 15071 - protein, 9 aa, synthetic construct
GGAGTDTLQ

SEQ ID NO: 15072 - protein, 9 aa, synthetic construct
GGYGHDVLN

SEQ ID NO: 15073 - protein, 9 aa, synthetic construct
GGDGDDWVT

SEQ ID NO: 15074 - protein, 9 aa, synthetic construct
GGAGDDAVG

SEQ ID NO: 15075 - protein, 9 aa, synthetic construct
GGMGDDILT

SEQ ID NO: 15076 - protein, 9 aa, synthetic construct
GGVGPDTLR

SEQ ID NO: 15077 - protein, 9 aa, synthetic construct
GGAGTDTLW

SEQ ID NO: 15078 - protein, 9 aa, synthetic construct
GGPGSDALR

SEQ ID NO: 15079 - protein, 9 aa, synthetic construct
GGPGSDALF

SEQ ID NO: 15080 - protein, 9 aa, synthetic construct
GGYGDDVVH

SEQ ID NO: 15081 - protein, 9 aa, synthetic construct
GGFGNDDLT

SEQ ID NO: 15082 - protein, 9 aa, synthetic construct
GGHGADTLR

SEQ ID NO: 15083 - protein, 9 aa, synthetic construct
GGDGVDQLY

SEQ ID NO: 15084 - protein, 9 aa, synthetic construct
GGGGKDILN

SEQ ID NO: 15085 - protein, 9 aa, synthetic construct
GGNGVDFLN

SEQ ID NO: 15086 - protein, 9 aa, synthetic construct
GGNGVDFLE

SEQ ID NO: 15087 - protein, 9 aa, synthetic construct
GGSGSDTAT

SEQ ID NO: 15088 - protein, 9 aa, synthetic construct
GGLGNDRLH

SEQ ID NO: 15089 - protein, 9 aa, synthetic construct
GGPGNDRMF

SEQ ID NO: 15090 - protein, 9 aa, synthetic construct
GGAGADVYQ

SEQ ID NO: 15091 - protein, 9 aa, synthetic construct
GGDGIDSAV

SEQ ID NO: 15092 - protein, 9 aa, synthetic construct
GGPGNDRML

SEQ ID NO: 15093 - protein, 9 aa, synthetic construct
GGNGVDELH

SEQ ID NO: 15094 - protein, 9 aa, synthetic construct
GGHGADILS

SEQ ID NO: 15095 - protein, 9 aa, synthetic construct
GGNGVDAVS

SEQ ID NO: 15096 - protein, 9 aa, synthetic construct
GGDGIDLLY

SEQ ID NO: 15097 - protein, 9 aa, synthetic construct
GGAGADKMT

SEQ ID NO: 15098 - protein, 9 aa, synthetic construct
GGDGADHLD

SEQ ID NO: 15099 - protein, 9 aa, synthetic construct
GGMGDDMLF

SEQ ID NO: 15100 - protein, 9 aa, synthetic construct
GGDGADHIY

SEQ ID NO: 15101 - protein, 9 aa, synthetic construct
GGNGVDKIV

SEQ ID NO: 15102 - protein, 9 aa, synthetic construct
GGPGNDRLS

SEQ ID NO: 15103 - protein, 9 aa, synthetic construct
GGAGADVVY

SEQ ID NO: 15104 - protein, 9 aa, synthetic construct
GGEGDDVMT

SEQ ID NO: 15105 - protein, 9 aa, synthetic construct
GGPGNDRLF

SEQ ID NO: 15106 - protein, 9 aa, synthetic construct
GGVGSDVLV

SEQ ID NO: 15107 - protein, 9 aa, synthetic construct
GGDGADHIN

SEQ ID NO: 15108 - protein, 9 aa, synthetic construct
GGAGADVVS

SEQ ID NO: 15109 - protein, 9 aa, synthetic construct
GGGGDDVYI

SEQ ID NO: 15110 - protein, 9 aa, synthetic construct
GGVGSDYLD

SEQ ID NO: 15111 - protein, 9 aa, synthetic construct
GGSGSDDLY

SEQ ID NO: 15112 - protein, 9 aa, synthetic construct
GGEGDDIIF

SEQ ID NO: 15113 - protein, 9 aa, synthetic construct
GGGGTDRLD

SEQ ID NO: 15114 - protein, 9 aa, synthetic construct
GGKGADTID

SEQ ID NO: 15115 - protein, 9 aa, synthetic construct
GGDGADHLT

SEQ ID NO: 15116 - protein, 9 aa, synthetic construct
GGAGADKMN

SEQ ID NO: 15117 - protein, 9 aa, synthetic construct
GGNGTDYLE

SEQ ID NO: 15118 - protein, 9 aa, synthetic construct
GGSGSDTFR

SEQ ID NO: 15119 - protein, 9 aa, synthetic construct
GGEGDDKLH

SEQ ID NO: 15120 - protein, 9 aa, synthetic construct
GGSGSDTIK

SEQ ID NO: 15121 - protein, 9 aa, synthetic construct
GGVGSDTIS

SEQ ID NO: 15122 - protein, 9 aa, synthetic construct
GGVGSDTIY

SEQ ID NO: 15123 - protein, 9 aa, synthetic construct
GGNGTDTLM

SEQ ID NO: 15124 - protein, 9 aa, synthetic construct
GGKGDDSLH

SEQ ID NO: 15125 - protein, 9 aa, synthetic construct
GGDGHDMIG

SEQ ID NO: 15126 - protein, 9 aa, synthetic construct
GGFGNDELY

SEQ ID NO: 15127 - protein, 9 aa, synthetic construct
GGAGKDSYD

SEQ ID NO: 15128 - protein, 9 aa, synthetic construct
GGPGNDSLT

SEQ ID NO: 15129 - protein, 9 aa, synthetic construct
GGPGNDSLS

SEQ ID NO: 15130 - protein, 9 aa, synthetic construct
GGNGTDTLY

SEQ ID NO: 15131 - protein, 9 aa, synthetic construct
GGAGVDKFV

SEQ ID NO: 15132 - protein, 9 aa, synthetic construct
GGSGSDTIE

SEQ ID NO: 15133 - protein, 9 aa, synthetic construct
GGSGSDTFQ

SEQ ID NO: 15134 - protein, 9 aa, synthetic construct
GGDGNDWLK

SEQ ID NO: 15135 - protein, 9 aa, synthetic construct
GGLGKDTLV

SEQ ID NO: 15136 - protein, 9 aa, synthetic construct
GGVGSDTLN

SEQ ID NO: 15137 - protein, 9 aa, synthetic construct
GGNGTDTVT

SEQ ID NO: 15138 - protein, 9 aa, synthetic construct
GGYGDDSLI

SEQ ID NO: 15139 - protein, 9 aa, synthetic construct
GGDGADWLA

SEQ ID NO: 15140 - protein, 9 aa, synthetic construct
GGAGADWFD

SEQ ID NO: 15141 - protein, 9 aa, synthetic construct
GGAGVDKIL

SEQ ID NO: 15142 - protein, 9 aa, synthetic construct
GGPGNDSIG

SEQ ID NO: 15143 - protein, 9 aa, synthetic construct
GGAGVDKLA

SEQ ID NO: 15144 - protein, 9 aa, synthetic construct
GGEGDDNLA

SEQ ID NO: 15145 - protein, 9 aa, synthetic construct
GGGGKDVLD

SEQ ID NO: 15146 - protein, 9 aa, synthetic construct
GGGGSDGLV

SEQ ID NO: 15147 - protein, 9 aa, synthetic construct
GGAGADKMI

SEQ ID NO: 15148 - protein, 9 aa, synthetic construct
GGDGADHMV

SEQ ID NO: 15149 - protein, 9 aa, synthetic construct
GGNGVDLVS

SEQ ID NO: 15150 - protein, 9 aa, synthetic construct
GGDGADHFF

SEQ ID NO: 15151 - protein, 9 aa, synthetic construct
GGDGDDLVY

SEQ ID NO: 15152 - protein, 9 aa, synthetic construct
GGGGKDTLV

SEQ ID NO: 15153 - protein, 9 aa, synthetic construct
GGAGLDLVS

SEQ ID NO: 15154 - protein, 9 aa, synthetic construct
GGNGVDTLI

SEQ ID NO: 15155 - protein, 9 aa, synthetic construct
GGAGVDMLL

SEQ ID NO: 15156 - protein, 9 aa, synthetic construct
GGLGQDNMT

SEQ ID NO: 15157 - protein, 9 aa, synthetic construct
GGNGNDKIF

SEQ ID NO: 15158 - protein, 9 aa, synthetic construct
GGMGHDRLN

SEQ ID NO: 15159 - protein, 9 aa, synthetic construct
GGLGNDRIA

SEQ ID NO: 15160 - protein, 9 aa, synthetic construct
GGYGDDLLT

SEQ ID NO: 15161 - protein, 9 aa, synthetic construct
GGEGDDIIT

SEQ ID NO: 15162 - protein, 9 aa, synthetic construct
GGAGVDMLN

SEQ ID NO: 15163 - protein, 9 aa, synthetic construct
GGGGEDTLI

SEQ ID NO: 15164 - protein, 9 aa, synthetic construct
GGNGVDTLY

SEQ ID NO: 15165 - protein, 9 aa, synthetic construct
GGNGVDTVD

SEQ ID NO: 15166 - protein, 9 aa, synthetic construct
GGDGEDWLY

SEQ ID NO: 15167 - protein, 9 aa, synthetic construct
GGPGNDKLI

SEQ ID NO: 15168 - protein, 9 aa, synthetic construct
GGSGNDTVA

SEQ ID NO: 15169 - protein, 9 aa, synthetic construct
GGNGNDRIL

SEQ ID NO: 15170 - protein, 9 aa, synthetic construct
GGEGDDRFL

SEQ ID NO: 15171 - protein, 9 aa, synthetic construct
GGYGDDLLS

SEQ ID NO: 15172 - protein, 9 aa, synthetic construct
GGGGTDRLS

SEQ ID NO: 15173 - protein, 9 aa, synthetic construct
GGLGNDRFS

SEQ ID NO: 15174 - protein, 9 aa, synthetic construct
GGEGRDLLE

SEQ ID NO: 15175 - protein, 9 aa, synthetic construct
GGAGLDMAA

SEQ ID NO: 15176 - protein, 9 aa, synthetic construct
GGDGIDIAS

SEQ ID NO: 15177 - protein, 9 aa, synthetic construct
GGPGNDIYR

SEQ ID NO: 15178 - protein, 9 aa, synthetic construct
GGYGDDLLF

SEQ ID NO: 15179 - protein, 9 aa, synthetic construct
GGEGDDKLD

SEQ ID NO: 15180 - protein, 9 aa, synthetic construct
GGYGDDLLE

SEQ ID NO: 15181 - protein, 9 aa, synthetic construct
GGSGSDSID

SEQ ID NO: 15182 - protein, 9 aa, synthetic construct
GGDGADFLH

SEQ ID NO: 15183 - protein, 9 aa, synthetic construct
GGGGYDYVY

SEQ ID NO: 15184 - protein, 9 aa, synthetic construct
GGYGDDNLD

SEQ ID NO: 15185 - protein, 9 aa, synthetic construct
GGLGKDVLS

SEQ ID NO: 15186 - protein, 9 aa, synthetic construct
GGDGNDWLR

SEQ ID NO: 15187 - protein, 9 aa, synthetic construct
GGEGDDNLF

SEQ ID NO: 15188 - protein, 9 aa, synthetic construct
GGGGDDVVL

SEQ ID NO: 15189 - protein, 9 aa, synthetic construct
GGDGADWID

SEQ ID NO: 15190 - protein, 9 aa, synthetic construct
GGLGNDRIY

SEQ ID NO: 15191 - protein, 9 aa, synthetic construct
GGAGVDLLA

SEQ ID NO: 15192 - protein, 9 aa, synthetic construct
GGAGADVMY

SEQ ID NO: 15193 - protein, 9 aa, synthetic construct
GGSGNDTME

SEQ ID NO: 15194 - protein, 9 aa, synthetic construct
GGDGEDTLW

SEQ ID NO: 15195 - protein, 9 aa, synthetic construct
GGDGNDYMN

SEQ ID NO: 15196 - protein, 9 aa, synthetic construct
GGMGHDTLK

SEQ ID NO: 15197 - protein, 9 aa, synthetic construct
GGAGLDTME

SEQ ID NO: 15198 - protein, 9 aa, synthetic construct
GGPGNDMLY

SEQ ID NO: 15199 - protein, 9 aa, synthetic construct
GGDGIDLIV

SEQ ID NO: 15200 - protein, 9 aa, synthetic construct
GGKGDDVYM

SEQ ID NO: 15201 - protein, 9 aa, synthetic construct
GGYGDDQLE

SEQ ID NO: 15202 - protein, 9 aa, synthetic construct
GGEGDDIIL

SEQ ID NO: 15203 - protein, 9 aa, synthetic construct
GGAGVDLLY

SEQ ID NO: 15204 - protein, 9 aa, synthetic construct
GGEGEDAIF

SEQ ID NO: 15205 - protein, 9 aa, synthetic construct
GGEGDDRIW

SEQ ID NO: 15206 - protein, 9 aa, synthetic construct
GGKGADTIT

SEQ ID NO: 15207 - protein, 9 aa, synthetic construct
GGPGNDLLV

SEQ ID NO: 15208 - protein, 9 aa, synthetic construct
GGAGKDLFV

SEQ ID NO: 15209 - protein, 9 aa, synthetic construct
GGPGNDLLM

SEQ ID NO: 15210 - protein, 9 aa, synthetic construct
GGEGDDLIA

SEQ ID NO: 15211 - protein, 9 aa, synthetic construct
GGSGSDSIN

SEQ ID NO: 15212 - protein, 9 aa, synthetic construct
GGHGADDID

SEQ ID NO: 15213 - protein, 9 aa, synthetic construct
GGNGNDIYY

SEQ ID NO: 15214 - protein, 9 aa, synthetic construct
GGGGDDLVT

SEQ ID NO: 15215 - protein, 9 aa, synthetic construct
GGNGDDTIT

SEQ ID NO: 15216 - protein, 9 aa, synthetic construct
GGLGLDHYD

SEQ ID NO: 15217 - protein, 9 aa, synthetic construct
GGPGNDTAN

SEQ ID NO: 15218 - protein, 9 aa, synthetic construct
GGYGDDTII

SEQ ID NO: 15219 - protein, 9 aa, synthetic construct
GGYGDDTIQ

SEQ ID NO: 15220 - protein, 9 aa, synthetic construct
GGSGSDTVQ

SEQ ID NO: 15221 - protein, 9 aa, synthetic construct
GGKGDDSAN

SEQ ID NO: 15222 - protein, 9 aa, synthetic construct
GGNGSDYLA

SEQ ID NO: 15223 - protein, 9 aa, synthetic construct
GGAGKDTFD

SEQ ID NO: 15224 - protein, 9 aa, synthetic construct
GGPGNDYIE

SEQ ID NO: 15225 - protein, 9 aa, synthetic construct
GGPGNDYID

SEQ ID NO: 15226 - protein, 9 aa, synthetic construct
GGGGDDWLT

SEQ ID NO: 15227 - protein, 9 aa, synthetic construct
GGPGNDWVL

SEQ ID NO: 15228 - protein, 9 aa, synthetic construct
GGSGQDQLT

SEQ ID NO: 15229 - protein, 9 aa, synthetic construct
GGGGKDVLY

SEQ ID NO: 15230 - protein, 9 aa, synthetic construct
GGGGDDLFL

SEQ ID NO: 15231 - protein, 9 aa, synthetic construct
GGEGEDVIS

SEQ ID NO: 15232 - protein, 9 aa, synthetic construct
GGGGKDVLV

SEQ ID NO: 15233 - protein, 9 aa, synthetic construct
GGGGIDVLY

SEQ ID NO: 15234 - protein, 9 aa, synthetic construct
GGPGNDVYY

SEQ ID NO: 15235 - protein, 9 aa, synthetic construct
GGLGKDRLT

SEQ ID NO: 15236 - protein, 9 aa, synthetic construct
GGGGDDWLY

SEQ ID NO: 15237 - protein, 9 aa, synthetic construct
GGLGSDRLD

SEQ ID NO: 15238 - protein, 9 aa, synthetic construct
GGLGKDRML

SEQ ID NO: 15239 - protein, 9 aa, synthetic construct
GGYGDDVLI

SEQ ID NO: 15240 - protein, 9 aa, synthetic construct
GGAGVDHLW

SEQ ID NO: 15241 - protein, 9 aa, synthetic construct
GGEGRDVLI

SEQ ID NO: 15242 - protein, 9 aa, synthetic construct
GGAGADYFD

SEQ ID NO: 15243 - protein, 9 aa, synthetic construct
GGDGNDTYR

SEQ ID NO: 15244 - protein, 9 aa, synthetic construct
GGLGNDSFI

SEQ ID NO: 15245 - protein, 9 aa, synthetic construct
GGGGDDLII

SEQ ID NO: 15246 - protein, 9 aa, synthetic construct
GGGGTDLIY

SEQ ID NO: 15247 - protein, 9 aa, synthetic construct
GGNGTDEMK

SEQ ID NO: 15248 - protein, 9 aa, synthetic construct
GGLGVDTLD

SEQ ID NO: 15249 - protein, 9 aa, synthetic construct
GGAGKDTFA

SEQ ID NO: 15250 - protein, 9 aa, synthetic construct
GGLGKDSLF

SEQ ID NO: 15251 - protein, 9 aa, synthetic construct
GGEGADLLS

SEQ ID NO: 15252 - protein, 9 aa, synthetic construct
GGSGNDTAY

SEQ ID NO: 15253 - protein, 9 aa, synthetic construct
GGDGVDLLV

SEQ ID NO: 15254 - protein, 9 aa, synthetic construct
GGGGTDKLF

SEQ ID NO: 15255 - protein, 9 aa, synthetic construct
GGAGVDDVA

SEQ ID NO: 15256 - protein, 9 aa, synthetic construct
GGLGKDKLI

SEQ ID NO: 15257 - protein, 9 aa, synthetic construct
GGNGDDNLQ

SEQ ID NO: 15258 - protein, 9 aa, synthetic construct
GGLGKDKLW

SEQ ID NO: 15259 - protein, 9 aa, synthetic construct
GGLGKDKLY

SEQ ID NO: 15260 - protein, 9 aa, synthetic construct
GGNGSDVLK

SEQ ID NO: 15261 - protein, 9 aa, synthetic construct
GGSGQDRLA

SEQ ID NO: 15262 - protein, 9 aa, synthetic construct
GGGGDDKLD

SEQ ID NO: 15263 - protein, 9 aa, synthetic construct
GGPGPDTLL

SEQ ID NO: 15264 - protein, 9 aa, synthetic construct
GGGGEDTLV

SEQ ID NO: 15265 - protein, 9 aa, synthetic construct
GGSGQDRFL

SEQ ID NO: 15266 - protein, 9 aa, synthetic construct
GGAGLDIVD

SEQ ID NO: 15267 - protein, 9 aa, synthetic construct
GGEGEDVLR

SEQ ID NO: 15268 - protein, 9 aa, synthetic construct
GGDGADKIN

SEQ ID NO: 15269 - protein, 9 aa, synthetic construct
GGLGNDSIS

SEQ ID NO: 15270 - protein, 9 aa, synthetic construct
GGEGDDRVR

SEQ ID NO: 15271 - protein, 9 aa, synthetic construct
GGNGNDIIW

SEQ ID NO: 15272 - protein, 9 aa, synthetic construct
GGNGSDVLY

SEQ ID NO: 15273 - protein, 9 aa, synthetic construct
GGNGSDVMH

SEQ ID NO: 15274 - protein, 9 aa, synthetic construct
GGGGSDIAV

SEQ ID NO: 15275 - protein, 9 aa, synthetic construct
GGAGVDFAD

SEQ ID NO: 15276 - protein, 9 aa, synthetic construct
GGDGNDYVN

SEQ ID NO: 15277 - protein, 9 aa, synthetic construct
GGAGVDFLA

SEQ ID NO: 15278 - protein, 9 aa, synthetic construct
GGNGSDVVT

SEQ ID NO: 15279 - protein, 9 aa, synthetic construct
GGSGSDTYF

SEQ ID NO: 15280 - protein, 9 aa, synthetic construct
GGYGDDVLV

SEQ ID NO: 15281 - protein, 9 aa, synthetic construct
GGDGADKFV

SEQ ID NO: 15282 - protein, 9 aa, synthetic construct
GGYGDDVLS

SEQ ID NO: 15283 - protein, 9 aa, synthetic construct
GGHGADTLD

SEQ ID NO: 15284 - protein, 9 aa, synthetic construct
GGLGKDQID

SEQ ID NO: 15285 - protein, 9 aa, synthetic construct
GGPGNDVLR

SEQ ID NO: 15286 - protein, 9 aa, synthetic construct
GGLGNDSFF

SEQ ID NO: 15287 - protein, 9 aa, synthetic construct
GGAGVDIMR

SEQ ID NO: 15288 - protein, 9 aa, synthetic construct
GGVGSDSMI

SEQ ID NO: 15289 - protein, 9 aa, synthetic construct
GGDGNDWLF

SEQ ID NO: 15290 - protein, 9 aa, synthetic construct
GGVGSDRLT

SEQ ID NO: 15291 - protein, 9 aa, synthetic construct
GGSGNDTIQ

SEQ ID NO: 15292 - protein, 9 aa, synthetic construct
GGEGRDTYI

SEQ ID NO: 15293 - protein, 9 aa, synthetic construct
GGVGSDRYE

SEQ ID NO: 15294 - protein, 9 aa, synthetic construct
GGAGVDILR

SEQ ID NO: 15295 - protein, 9 aa, synthetic construct
GGGGKDIFD

SEQ ID NO: 15296 - protein, 9 aa, synthetic construct
GGDGFDVML

SEQ ID NO: 15297 - protein, 9 aa, synthetic construct
GGNGTDRLT

SEQ ID NO: 15298 - protein, 9 aa, synthetic construct
GGVGSDSLI

SEQ ID NO: 15299 - protein, 9 aa, synthetic construct
GGNGNDRLK

SEQ ID NO: 15300 - protein, 9 aa, synthetic construct
GGPGNDTLG

SEQ ID NO: 15301 - protein, 9 aa, synthetic construct
GGYGDDTLF

SEQ ID NO: 15302 - protein, 9 aa, synthetic construct
GGEGDDKLL

SEQ ID NO: 15303 - protein, 9 aa, synthetic construct
GGFGNDELL

SEQ ID NO: 15304 - protein, 9 aa, synthetic construct
GGNGTDRAV

SEQ ID NO: 15305 - protein, 9 aa, synthetic construct
GGSGSDTIV

SEQ ID NO: 15306 - protein, 9 aa, synthetic construct
GGFGNDELR

SEQ ID NO: 15307 - protein, 9 aa, synthetic construct
GGDGADWLD

SEQ ID NO: 15308 - protein, 9 aa, synthetic construct
GGPGNDTIT

SEQ ID NO: 15309 - protein, 9 aa, synthetic construct
GGLGNDRMV

SEQ ID NO: 15310 - protein, 9 aa, synthetic construct
GGAGVDILT

SEQ ID NO: 15311 - protein, 9 aa, synthetic construct
GGMGIDLVF

SEQ ID NO: 15312 - protein, 9 aa, synthetic construct
GGEGRDTVD

SEQ ID NO: 15313 - protein, 9 aa, synthetic construct
GGAGKDKLN

SEQ ID NO: 15314 - protein, 9 aa, synthetic construct
GGEGDDKLK

SEQ ID NO: 15315 - protein, 9 aa, synthetic construct
GGNGTDTAV

SEQ ID NO: 15316 - protein, 9 aa, synthetic construct
GGPGNDTIF

SEQ ID NO: 15317 - protein, 9 aa, synthetic construct
GGDGADIIH

SEQ ID NO: 15318 - protein, 9 aa, synthetic construct
GGVGSDTFV

SEQ ID NO: 15319 - protein, 9 aa, synthetic construct
GGHGADRLS

SEQ ID NO: 15320 - protein, 9 aa, synthetic construct
GGLGQDRLV

SEQ ID NO: 15321 - protein, 9 aa, synthetic construct
GGGGHDMLI

SEQ ID NO: 15322 - protein, 9 aa, synthetic construct
GGPGNDVIF

SEQ ID NO: 15323 - protein, 9 aa, synthetic construct
GGDGADIME

SEQ ID NO: 15324 - protein, 9 aa, synthetic construct
GGSGSDTVD

SEQ ID NO: 15325 - protein, 9 aa, synthetic construct
GGLGKDSLL

SEQ ID NO: 15326 - protein, 9 aa, synthetic construct
GGSGRDYLW

SEQ ID NO: 15327 - protein, 9 aa, synthetic construct
GGAGADWVR

SEQ ID NO: 15328 - protein, 9 aa, synthetic construct
GGGGSDHLF

SEQ ID NO: 15329 - protein, 9 aa, synthetic construct
GGDGYDRLN

SEQ ID NO: 15330 - protein, 9 aa, synthetic construct
GGLGNDSFE

SEQ ID NO: 15331 - protein, 9 aa, synthetic construct
GGGGTDLLT

SEQ ID NO: 15332 - protein, 9 aa, synthetic construct
GGPGNDVIT

SEQ ID NO: 15333 - protein, 9 aa, synthetic construct
GGAGADWMN

SEQ ID NO: 15334 - protein, 9 aa, synthetic construct
GGYGDDTVS

SEQ ID NO: 15335 - protein, 9 aa, synthetic construct
GGDGNDWLA

SEQ ID NO: 15336 - protein, 9 aa, synthetic construct
GGLGKDTFT

SEQ ID NO: 15337 - protein, 9 aa, synthetic construct
GGEGRDVFF

SEQ ID NO: 15338 - protein, 9 aa, synthetic construct
GGDGNDTYT

SEQ ID NO: 15339 - protein, 9 aa, synthetic construct
GGAGVDIIN

SEQ ID NO: 15340 - protein, 9 aa, synthetic construct
GGSGSDTMS

SEQ ID NO: 15341 - protein, 9 aa, synthetic construct
GGLGPDLLV

SEQ ID NO: 15342 - protein, 9 aa, synthetic construct
GGDGADILL

SEQ ID NO: 15343 - protein, 9 aa, synthetic construct
GGEGADLLQ

SEQ ID NO: 15344 - protein, 9 aa, synthetic construct
GGSGQDQFL

SEQ ID NO: 15345 - protein, 9 aa, synthetic construct
GGKGADTFI

SEQ ID NO: 15346 - protein, 9 aa, synthetic construct
GGAGADWLY

SEQ ID NO: 15347 - protein, 9 aa, synthetic construct
GGPGNDTMV

SEQ ID NO: 15348 - protein, 9 aa, synthetic construct
GGAGADKIT

SEQ ID NO: 15349 - protein, 9 aa, synthetic construct
GGGGTDLLY

SEQ ID NO: 15350 - protein, 9 aa, synthetic construct
GGKGADTFM

SEQ ID NO: 15351 - protein, 9 aa, synthetic construct
GGDGHDLLK

SEQ ID NO: 15352 - protein, 9 aa, synthetic construct
GGLGKDTIY

SEQ ID NO: 15353 - protein, 9 aa, synthetic construct
GGTGDDHLT

SEQ ID NO: 15354 - protein, 9 aa, synthetic construct
GGGGADTFG

SEQ ID NO: 15355 - protein, 9 aa, synthetic construct
GGAGSDVIE

SEQ ID NO: 15356 - protein, 9 aa, synthetic construct
GGSGADALH

SEQ ID NO: 15357 - protein, 9 aa, synthetic construct
GGKGSDSLT

SEQ ID NO: 15358 - protein, 9 aa, synthetic construct
GGKGSDSLE

SEQ ID NO: 15359 - protein, 9 aa, synthetic construct
GGTGNDFMQ

SEQ ID NO: 15360 - protein, 9 aa, synthetic construct
GGTGNDFMG

SEQ ID NO: 15361 - protein, 9 aa, synthetic construct
GGSGADAMS

SEQ ID NO: 15362 - protein, 9 aa, synthetic construct
GGSGADAMW

SEQ ID NO: 15363 - protein, 9 aa, synthetic construct
GGTGNDFME

SEQ ID NO: 15364 - protein, 9 aa, synthetic construct
GGTGNDFLY

SEQ ID NO: 15365 - protein, 9 aa, synthetic construct
GGKGSDRMI

SEQ ID NO: 15366 - protein, 9 aa, synthetic construct
GGSGADDFV

SEQ ID NO: 15367 - protein, 9 aa, synthetic construct
GGDGNDKLL

SEQ ID NO: 15368 - protein, 9 aa, synthetic construct
GGSGADDIG

SEQ ID NO: 15369 - protein, 9 aa, synthetic construct
GGAGNDWIK

SEQ ID NO: 15370 - protein, 9 aa, synthetic construct
GGSGADDIK

SEQ ID NO: 15371 - protein, 9 aa, synthetic construct
GGNGADRLN

SEQ ID NO: 15372 - protein, 9 aa, synthetic construct
GGFGTDTLY

SEQ ID NO: 15373 - protein, 9 aa, synthetic construct
GGSGADDIS

SEQ ID NO: 15374 - protein, 9 aa, synthetic construct
GGDGSDFVN

SEQ ID NO: 15375 - protein, 9 aa, synthetic construct
GGKGSDRLE

SEQ ID NO: 15376 - protein, 9 aa, synthetic construct
GGTGADQLD

SEQ ID NO: 15377 - protein, 9 aa, synthetic construct
GGIGGDTIT

SEQ ID NO: 15378 - protein, 9 aa, synthetic construct
GGTGNDHLW

SEQ ID NO: 15379 - protein, 9 aa, synthetic construct
GGSGADALA

SEQ ID NO: 15380 - protein, 9 aa, synthetic construct
GGTGNDHLS

SEQ ID NO: 15381 - protein, 9 aa, synthetic construct
GGTGADQIS

SEQ ID NO: 15382 - protein, 9 aa, synthetic construct
GGTGNDHLL

SEQ ID NO: 15383 - protein, 9 aa, synthetic construct
GGRGWDRLY

SEQ ID NO: 15384 - protein, 9 aa, synthetic construct
GGTGNDHLI

SEQ ID NO: 15385 - protein, 9 aa, synthetic construct
GGAGNDFYL

SEQ ID NO: 15386 - protein, 9 aa, synthetic construct
GGGGGDELY

SEQ ID NO: 15387 - protein, 9 aa, synthetic construct
GGAGNDFYY

SEQ ID NO: 15388 - protein, 9 aa, synthetic construct
GGNGADRIT

SEQ ID NO: 15389 - protein, 9 aa, synthetic construct
GGTGNDHLD

SEQ ID NO: 15390 - protein, 9 aa, synthetic construct
GGDGNDKIL

SEQ ID NO: 15391 - protein, 9 aa, synthetic construct
GGDGFDRLF

SEQ ID NO: 15392 - protein, 9 aa, synthetic construct
GGTGNDGLS

SEQ ID NO: 15393 - protein, 9 aa, synthetic construct
GGAGNDWLG

SEQ ID NO: 15394 - protein, 9 aa, synthetic construct
GGAGNDGFI

SEQ ID NO: 15395 - protein, 9 aa, synthetic construct
GGTGNDGLN

SEQ ID NO: 15396 - protein, 9 aa, synthetic construct
GGSGADAFR

SEQ ID NO: 15397 - protein, 9 aa, synthetic construct
GGEGKDKLY

SEQ ID NO: 15398 - protein, 9 aa, synthetic construct
GGTGNDFVL

SEQ ID NO: 15399 - protein, 9 aa, synthetic construct
GGNGDDVMI

SEQ ID NO: 15400 - protein, 9 aa, synthetic construct
GGTGADQLH

SEQ ID NO: 15401 - protein, 9 aa, synthetic construct
GGSGIDTAA

SEQ ID NO: 15402 - protein, 9 aa, synthetic construct
GGTGNDFIG

SEQ ID NO: 15403 - protein, 9 aa, synthetic construct
GGIGHDLID

SEQ ID NO: 15404 - protein, 9 aa, synthetic construct
GGTGADQLR

SEQ ID NO: 15405 - protein, 9 aa, synthetic construct
GGAGFDRVD

SEQ ID NO: 15406 - protein, 9 aa, synthetic construct
GGDGSDEVI

SEQ ID NO: 15407 - protein, 9 aa, synthetic construct
GGKGSDLID

SEQ ID NO: 15408 - protein, 9 aa, synthetic construct
GGTGNDDMG

SEQ ID NO: 15409 - protein, 9 aa, synthetic construct
GGKGKDYIE

SEQ ID NO: 15410 - protein, 9 aa, synthetic construct
GGSGADFLS

SEQ ID NO: 15411 - protein, 9 aa, synthetic construct
GGTGNDDME

SEQ ID NO: 15412 - protein, 9 aa, synthetic construct
GGTGNDDMD

SEQ ID NO: 15413 - protein, 9 aa, synthetic construct
GGSGADFVI

SEQ ID NO: 15414 - protein, 9 aa, synthetic construct
GGAGNDVVI

SEQ ID NO: 15415 - protein, 9 aa, synthetic construct
GGNGDDVVN

SEQ ID NO: 15416 - protein, 9 aa, synthetic construct
GGIGSDTID

SEQ ID NO: 15417 - protein, 9 aa, synthetic construct
GGTGADQMA

SEQ ID NO: 15418 - protein, 9 aa, synthetic construct
GGEGVDTAV

SEQ ID NO: 15419 - protein, 9 aa, synthetic construct
GGSGADHFY

SEQ ID NO: 15420 - protein, 9 aa, synthetic construct
GGEGNDQLC

SEQ ID NO: 15421 - protein, 9 aa, synthetic construct
GGIGHDRLA

SEQ ID NO: 15422 - protein, 9 aa, synthetic construct
GGDGSDFAL

SEQ ID NO: 15423 - protein, 9 aa, synthetic construct
GGAGNDVYE

SEQ ID NO: 15424 - protein, 9 aa, synthetic construct
GGAGFDRMI

SEQ ID NO: 15425 - protein, 9 aa, synthetic construct
GGAGNDVYW

SEQ ID NO: 15426 - protein, 9 aa, synthetic construct
GGAGNDWFW

SEQ ID NO: 15427 - protein, 9 aa, synthetic construct
GGTGNDFIE

SEQ ID NO: 15428 - protein, 9 aa, synthetic construct
GGAGFDRFT

SEQ ID NO: 15429 - protein, 9 aa, synthetic construct
GGNGADRMK

SEQ ID NO: 15430 - protein, 9 aa, synthetic construct
GGDGSDFLN

SEQ ID NO: 15431 - protein, 9 aa, synthetic construct
GGKGKDVMT

SEQ ID NO: 15432 - protein, 9 aa, synthetic construct
GGNGGDDMM

SEQ ID NO: 15433 - protein, 9 aa, synthetic construct
GGSGADEIH

SEQ ID NO: 15434 - protein, 9 aa, synthetic construct
GGSGADELD

SEQ ID NO: 15435 - protein, 9 aa, synthetic construct
GGTGNDEIF

SEQ ID NO: 15436 - protein, 9 aa, synthetic construct
GGTGNDELR

SEQ ID NO: 15437 - protein, 9 aa, synthetic construct
GGDGGDLLT

SEQ ID NO: 15438 - protein, 9 aa, synthetic construct
GGAGNDVYK

SEQ ID NO: 15439 - protein, 9 aa, synthetic construct
GGDGDDSLG

SEQ ID NO: 15440 - protein, 9 aa, synthetic construct
GGNGGDALY

SEQ ID NO: 15441 - protein, 9 aa, synthetic construct
GGEGADTAL

SEQ ID NO: 15442 - protein, 9 aa, synthetic construct
GGNGGDALN

SEQ ID NO: 15443 - protein, 9 aa, synthetic construct
GGAGNDVYF

SEQ ID NO: 15444 - protein, 9 aa, synthetic construct
GGSGIDTIY

SEQ ID NO: 15445 - protein, 9 aa, synthetic construct
GGTGNDHLY

SEQ ID NO: 15446 - protein, 9 aa, synthetic construct
GGDGDDHVS

SEQ ID NO: 15447 - protein, 9 aa, synthetic construct
GGIGSDTLV

SEQ ID NO: 15448 - protein, 9 aa, synthetic construct
GGEGNDGLM

SEQ ID NO: 15449 - protein, 9 aa, synthetic construct
GGIGFDLLQ

SEQ ID NO: 15450 - protein, 9 aa, synthetic construct
GGAGNDYVF

SEQ ID NO: 15451 - protein, 9 aa, synthetic construct
GGNGADQLF

SEQ ID NO: 15452 - protein, 9 aa, synthetic construct
GGAGNDYVA

SEQ ID NO: 15453 - protein, 9 aa, synthetic construct
GGNGADQLL

SEQ ID NO: 15454 - protein, 9 aa, synthetic construct
GGTGNDKID

SEQ ID NO: 15455 - protein, 9 aa, synthetic construct
GGTGADNMN

SEQ ID NO: 15456 - protein, 9 aa, synthetic construct
GGAGNDYML

SEQ ID NO: 15457 - protein, 9 aa, synthetic construct
GGKGKDTLS

SEQ ID NO: 15458 - protein, 9 aa, synthetic construct
GGKGSDVFV

SEQ ID NO: 15459 - protein, 9 aa, synthetic construct
GGAGNDYMF

SEQ ID NO: 15460 - protein, 9 aa, synthetic construct
GGIGFDSLD

SEQ ID NO: 15461 - protein, 9 aa, synthetic construct
GGRGTDILN

SEQ ID NO: 15462 - protein, 9 aa, synthetic construct
GGRGTDILT

SEQ ID NO: 15463 - protein, 9 aa, synthetic construct
GGTGNDIVV

SEQ ID NO: 15464 - protein, 9 aa, synthetic construct
GGKGSDVFI

SEQ ID NO: 15465 - protein, 9 aa, synthetic construct
GGAGNDYLR

SEQ ID NO: 15466 - protein, 9 aa, synthetic construct
GGGGQDLLM

SEQ ID NO: 15467 - protein, 9 aa, synthetic construct
GGTGNDKLA

SEQ ID NO: 15468 - protein, 9 aa, synthetic construct
GGDGNDIMR

SEQ ID NO: 15469 - protein, 9 aa, synthetic construct
GGEGADSMV

SEQ ID NO: 15470 - protein, 9 aa, synthetic construct
GGRGSDTYY

SEQ ID NO: 15471 - protein, 9 aa, synthetic construct
GGFGVDVLK

SEQ ID NO: 15472 - protein, 9 aa, synthetic construct
GGAGPDKVY

SEQ ID NO: 15473 - protein, 9 aa, synthetic construct
GGEGHDTVS

SEQ ID NO: 15474 - protein, 9 aa, synthetic construct
GGNGADQIG

SEQ ID NO: 15475 - protein, 9 aa, synthetic construct
GGFGDDQMW

SEQ ID NO: 15476 - protein, 9 aa, synthetic construct
GGEGNDRFF

SEQ ID NO: 15477 - protein, 9 aa, synthetic construct
GGRGSDTFI

SEQ ID NO: 15478 - protein, 9 aa, synthetic construct
GGRGSDTFV

SEQ ID NO: 15479 - protein, 9 aa, synthetic construct
GGIGEDVLS

SEQ ID NO: 15480 - protein, 9 aa, synthetic construct
GGDGNDILW

SEQ ID NO: 15481 - protein, 9 aa, synthetic construct
GGAGPDALF

SEQ ID NO: 15482 - protein, 9 aa, synthetic construct
GGFGNDVLV

SEQ ID NO: 15483 - protein, 9 aa, synthetic construct
GGFGVDRFT

SEQ ID NO: 15484 - protein, 9 aa, synthetic construct
GGDGDDIAS

SEQ ID NO: 15485 - protein, 9 aa, synthetic construct
GGAGFDILK

SEQ ID NO: 15486 - protein, 9 aa, synthetic construct
GGLGTDKLY

SEQ ID NO: 15487 - protein, 9 aa, synthetic construct
GGRGSDTVL

SEQ ID NO: 15488 - protein, 9 aa, synthetic construct
GGDGNDIMI

SEQ ID NO: 15489 - protein, 9 aa, synthetic construct
GGAGNDYYY

SEQ ID NO: 15490 - protein, 9 aa, synthetic construct
GGTGNDIMY

SEQ ID NO: 15491 - protein, 9 aa, synthetic construct
GGTGADNYY

SEQ ID NO: 15492 - protein, 9 aa, synthetic construct
GGGGQDLLL

SEQ ID NO: 15493 - protein, 9 aa, synthetic construct
GGTGNDIML

SEQ ID NO: 15494 - protein, 9 aa, synthetic construct
GGDGSDHLY

SEQ ID NO: 15495 - protein, 9 aa, synthetic construct
GGTGNDIAR

SEQ ID NO: 15496 - protein, 9 aa, synthetic construct
GGEGNDGLS

SEQ ID NO: 15497 - protein, 9 aa, synthetic construct
GGKGSDTLL

SEQ ID NO: 15498 - protein, 9 aa, synthetic construct
GGGGHDTLE

SEQ ID NO: 15499 - protein, 9 aa, synthetic construct
GGKGSDTLK

SEQ ID NO: 15500 - protein, 9 aa, synthetic construct
GGRGVDRVL

SEQ ID NO: 15501 - protein, 9 aa, synthetic construct
GGGGQDILT

SEQ ID NO: 15502 - protein, 9 aa, synthetic construct
GGAGIDELT

SEQ ID NO: 15503 - protein, 9 aa, synthetic construct
GGRGVDTFI

SEQ ID NO: 15504 - protein, 9 aa, synthetic construct
GGGGNDLMG

SEQ ID NO: 15505 - protein, 9 aa, synthetic construct
GGAGNDWVF

SEQ ID NO: 15506 - protein, 9 aa, synthetic construct
GGKGSDTLE

SEQ ID NO: 15507 - protein, 9 aa, synthetic construct
GGDGNDKIE

SEQ ID NO: 15508 - protein, 9 aa, synthetic construct
GGSGIDTLE

SEQ ID NO: 15509 - protein, 9 aa, synthetic construct
GGKGSDTIN

SEQ ID NO: 15510 - protein, 9 aa, synthetic construct
GGRGVDTLV

SEQ ID NO: 15511 - protein, 9 aa, synthetic construct
GGGGNDQIS

SEQ ID NO: 15512 - protein, 9 aa, synthetic construct
GGAGNDWMA

SEQ ID NO: 15513 - protein, 9 aa, synthetic construct
GGKGSDTLY

SEQ ID NO: 15514 - protein, 9 aa, synthetic construct
GGGGQDKIR

SEQ ID NO: 15515 - protein, 9 aa, synthetic construct
GGEGCDIAS

SEQ ID NO: 15516 - protein, 9 aa, synthetic construct
GGTGNDIIL

SEQ ID NO: 15517 - protein, 9 aa, synthetic construct
GGDGNDRVL

SEQ ID NO: 15518 - protein, 9 aa, synthetic construct
GGIGFDTLI

SEQ ID NO: 15519 - protein, 9 aa, synthetic construct
GGEGVDLLR

SEQ ID NO: 15520 - protein, 9 aa, synthetic construct
GGAGNDYIT

SEQ ID NO: 15521 - protein, 9 aa, synthetic construct
GGKGKDTVS

SEQ ID NO: 15522 - protein, 9 aa, synthetic construct
GGRGTDTLD

SEQ ID NO: 15523 - protein, 9 aa, synthetic construct
GGRGTDTLN

SEQ ID NO: 15524 - protein, 9 aa, synthetic construct
GGEGVDLLS

SEQ ID NO: 15525 - protein, 9 aa, synthetic construct
GGRGTDTLY

SEQ ID NO: 15526 - protein, 9 aa, synthetic construct
GGDGNDRVE

SEQ ID NO: 15527 - protein, 9 aa, synthetic construct
GGDGNDIVT

SEQ ID NO: 15528 - protein, 9 aa, synthetic construct
GGAGNDYIL

SEQ ID NO: 15529 - protein, 9 aa, synthetic construct
GGAGIDEMR

SEQ ID NO: 15530 - protein, 9 aa, synthetic construct
GGTGADQFR

SEQ ID NO: 15531 - protein, 9 aa, synthetic construct
GGTGNDIIF

SEQ ID NO: 15532 - protein, 9 aa, synthetic construct
GGSGIDTLR

SEQ ID NO: 15533 - protein, 9 aa, synthetic construct
GGAGFDLIL

SEQ ID NO: 15534 - protein, 9 aa, synthetic construct
GGIGGDALF

SEQ ID NO: 15535 - protein, 9 aa, synthetic construct
GGSGIDRFV

SEQ ID NO: 15536 - protein, 9 aa, synthetic construct
GGSGADHLV

SEQ ID NO: 15537 - protein, 9 aa, synthetic construct
GGAGNDVMM

SEQ ID NO: 15538 - protein, 9 aa, synthetic construct
GGLGTDALN

SEQ ID NO: 15539 - protein, 9 aa, synthetic construct
GGSGADQLD

SEQ ID NO: 15540 - protein, 9 aa, synthetic construct
GGSGADQLI

SEQ ID NO: 15541 - protein, 9 aa, synthetic construct
GGTGLDALY

SEQ ID NO: 15542 - protein, 9 aa, synthetic construct
GGAGFDYLH

SEQ ID NO: 15543 - protein, 9 aa, synthetic construct
GGFGDDLLT

SEQ ID NO: 15544 - protein, 9 aa, synthetic construct
GGDGDDQIA

SEQ ID NO: 15545 - protein, 9 aa, synthetic construct
GGKGNDAIY

SEQ ID NO: 15546 - protein, 9 aa, synthetic construct
GGEGADTIN

SEQ ID NO: 15547 - protein, 9 aa, synthetic construct
GGEGNDNLF

SEQ ID NO: 15548 - protein, 9 aa, synthetic construct
GGDGNDLLG

SEQ ID NO: 15549 - protein, 9 aa, synthetic construct
GGKGNDALD

SEQ ID NO: 15550 - protein, 9 aa, synthetic construct
GGSGIDAAY

SEQ ID NO: 15551 - protein, 9 aa, synthetic construct
GGIGKDVIN

SEQ ID NO: 15552 - protein, 9 aa, synthetic construct
GGAGGDAIN

SEQ ID NO: 15553 - protein, 9 aa, synthetic construct
GGEGWDRLV

SEQ ID NO: 15554 - protein, 9 aa, synthetic construct
GGSGHDYLY

SEQ ID NO: 15555 - protein, 9 aa, synthetic construct
GGTGKDVIY

SEQ ID NO: 15556 - protein, 9 aa, synthetic construct
GGKGRDTLI

SEQ ID NO: 15557 - protein, 9 aa, synthetic construct
GGDGGDLLE

SEQ ID NO: 15558 - protein, 9 aa, synthetic construct
GGSGADQLA

SEQ ID NO: 15559 - protein, 9 aa, synthetic construct
GGGGNDYMD

SEQ ID NO: 15560 - protein, 9 aa, synthetic construct
GGLGSDALE

SEQ ID NO: 15561 - protein, 9 aa, synthetic construct
GGDGDDSAH

SEQ ID NO: 15562 - protein, 9 aa, synthetic construct
GGAGNDVAW

SEQ ID NO: 15563 - protein, 9 aa, synthetic construct
GGTGLDMID

SEQ ID NO: 15564 - protein, 9 aa, synthetic construct
GGKGRDVLT

SEQ ID NO: 15565 - protein, 9 aa, synthetic construct
GGAGNDVAV

SEQ ID NO: 15566 - protein, 9 aa, synthetic construct
GGSGADMLI

SEQ ID NO: 15567 - protein, 9 aa, synthetic construct
GGSGADMLV

SEQ ID NO: 15568 - protein, 9 aa, synthetic construct
GGTGLDLLS

SEQ ID NO: 15569 - protein, 9 aa, synthetic construct
GGLGTDDVR

SEQ ID NO: 15570 - protein, 9 aa, synthetic construct
GGEGADTIF

SEQ ID NO: 15571 - protein, 9 aa, synthetic construct
GGAGNDVAA

SEQ ID NO: 15572 - protein, 9 aa, synthetic construct
GGAGNDHIV

SEQ ID NO: 15573 - protein, 9 aa, synthetic construct
GGDGRDWLY

SEQ ID NO: 15574 - protein, 9 aa, synthetic construct
GGKGMDYLD

SEQ ID NO: 15575 - protein, 9 aa, synthetic construct
GGSGADNLY

SEQ ID NO: 15576 - protein, 9 aa, synthetic construct
GGSGIDFAS

SEQ ID NO: 15577 - protein, 9 aa, synthetic construct
GGEGDDTFL

SEQ ID NO: 15578 - protein, 9 aa, synthetic construct
GGTGADRLR

SEQ ID NO: 15579 - protein, 9 aa, synthetic construct
GGEGADTIL

SEQ ID NO: 15580 - protein, 9 aa, synthetic construct
GGAGFDWLT

SEQ ID NO: 15581 - protein, 9 aa, synthetic construct
GGTGKDVFK

SEQ ID NO: 15582 - protein, 9 aa, synthetic construct
GGDGRDVLN

SEQ ID NO: 15583 - protein, 9 aa, synthetic construct
GGDGRDVLH

SEQ ID NO: 15584 - protein, 9 aa, synthetic construct
GGDGRDVLG

SEQ ID NO: 15585 - protein, 9 aa, synthetic construct
GGAGNDTMQ

SEQ ID NO: 15586 - protein, 9 aa, synthetic construct
GGTGKDRLE

SEQ ID NO: 15587 - protein, 9 aa, synthetic construct
GGSGADSFL

SEQ ID NO: 15588 - protein, 9 aa, synthetic construct
GGEGNDHLI

SEQ ID NO: 15589 - protein, 9 aa, synthetic construct
GGGGNDYLG

SEQ ID NO: 15590 - protein, 9 aa, synthetic construct
GGAGNDTMH

SEQ ID NO: 15591 - protein, 9 aa, synthetic construct
GGSGADSIK

SEQ ID NO: 15592 - protein, 9 aa, synthetic construct
GGSGADSIN

SEQ ID NO: 15593 - protein, 9 aa, synthetic construct
GGIGSDQLF

SEQ ID NO: 15594 - protein, 9 aa, synthetic construct
GGAGNDTMF

SEQ ID NO: 15595 - protein, 9 aa, synthetic construct
GGSGHDVLV

SEQ ID NO: 15596 - protein, 9 aa, synthetic construct
GGEGNDMLS

SEQ ID NO: 15597 - protein, 9 aa, synthetic construct
GGSGADSLH

SEQ ID NO: 15598 - protein, 9 aa, synthetic construct
GGAGGDELH

SEQ ID NO: 15599 - protein, 9 aa, synthetic construct
GGAGGDELR

SEQ ID NO: 15600 - protein, 9 aa, synthetic construct
GGEGYDILI

SEQ ID NO: 15601 - protein, 9 aa, synthetic construct
GGTGKDLLV

SEQ ID NO: 15602 - protein, 9 aa, synthetic construct
GGIGNDALT

SEQ ID NO: 15603 - protein, 9 aa, synthetic construct
GGEGNDMLM

SEQ ID NO: 15604 - protein, 9 aa, synthetic construct
GGIGSDRIF

SEQ ID NO: 15605 - protein, 9 aa, synthetic construct
GGSGADRVY

SEQ ID NO: 15606 - protein, 9 aa, synthetic construct
GGNGADTLF

SEQ ID NO: 15607 - protein, 9 aa, synthetic construct
GGSGHDWLY

SEQ ID NO: 15608 - protein, 9 aa, synthetic construct
GGSGADRIN

SEQ ID NO: 15609 - protein, 9 aa, synthetic construct
GGEGNDNIN

SEQ ID NO: 15610 - protein, 9 aa, synthetic construct
GGSGADRIV

SEQ ID NO: 15611 - protein, 9 aa, synthetic construct
GGKGNDALI

SEQ ID NO: 15612 - protein, 9 aa, synthetic construct
GGSGHDYLA

SEQ ID NO: 15613 - protein, 9 aa, synthetic construct
GGSGADRLH

SEQ ID NO: 15614 - protein, 9 aa, synthetic construct
GGTGKDTLN

SEQ ID NO: 15615 - protein, 9 aa, synthetic construct
GGTGADRMS

SEQ ID NO: 15616 - protein, 9 aa, synthetic construct
GGAGNDHLR

SEQ ID NO: 15617 - protein, 9 aa, synthetic construct
GGEGYDAVS

SEQ ID NO: 15618 - protein, 9 aa, synthetic construct
GGTGKDTLD

SEQ ID NO: 15619 - protein, 9 aa, synthetic construct
GGIGLDSFD

SEQ ID NO: 15620 - protein, 9 aa, synthetic construct
GGIGLDTLD

SEQ ID NO: 15621 - protein, 9 aa, synthetic construct
GGIGLDTLL

SEQ ID NO: 15622 - protein, 9 aa, synthetic construct
GGNGDDWIN

SEQ ID NO: 15623 - protein, 9 aa, synthetic construct
GGIGSDRIQ

SEQ ID NO: 15624 - protein, 9 aa, synthetic construct
GGAGGDDLD

SEQ ID NO: 15625 - protein, 9 aa, synthetic construct
GGAGGDDLL

SEQ ID NO: 15626 - protein, 9 aa, synthetic construct
GGAGNDHIN

SEQ ID NO: 15627 - protein, 9 aa, synthetic construct
GGDGRDYIE

SEQ ID NO: 15628 - protein, 9 aa, synthetic construct
GGAGNDVFE

SEQ ID NO: 15629 - protein, 9 aa, synthetic construct
GGSGADKMS

SEQ ID NO: 15630 - protein, 9 aa, synthetic construct
GGNGDDHLD

SEQ ID NO: 15631 - protein, 9 aa, synthetic construct
GGSGADIMA

SEQ ID NO: 15632 - protein, 9 aa, synthetic construct
GGSGADIMI

SEQ ID NO: 15633 - protein, 9 aa, synthetic construct
GGKGSDILD

SEQ ID NO: 15634 - protein, 9 aa, synthetic construct
GGTGNDAIS

SEQ ID NO: 15635 - protein, 9 aa, synthetic construct
GGIGHDTLI

SEQ ID NO: 15636 - protein, 9 aa, synthetic construct
GGAGFDTAN

SEQ ID NO: 15637 - protein, 9 aa, synthetic construct
GGTGNDAIH

SEQ ID NO: 15638 - protein, 9 aa, synthetic construct
GGIGHDTLL

SEQ ID NO: 15639 - protein, 9 aa, synthetic construct
GGKGSDIFI

SEQ ID NO: 15640 - protein, 9 aa, synthetic construct
GGTGMDYVS

SEQ ID NO: 15641 - protein, 9 aa, synthetic construct
GGNGDDHII

SEQ ID NO: 15642 - protein, 9 aa, synthetic construct
GGDGNDLFV

SEQ ID NO: 15643 - protein, 9 aa, synthetic construct
GGSGADKLL

SEQ ID NO: 15644 - protein, 9 aa, synthetic construct
GGTGADRFE

SEQ ID NO: 15645 - protein, 9 aa, synthetic construct
GGTGADRFF

SEQ ID NO: 15646 - protein, 9 aa, synthetic construct
GGAGFDTII

SEQ ID NO: 15647 - protein, 9 aa, synthetic construct
GGIGSDSLN

SEQ ID NO: 15648 - protein, 9 aa, synthetic construct
GGAGFDTIT

SEQ ID NO: 15649 - protein, 9 aa, synthetic construct
GGSGIDQLF

SEQ ID NO: 15650 - protein, 9 aa, synthetic construct
GGSGADILS

SEQ ID NO: 15651 - protein, 9 aa, synthetic construct
GGTGNDALV

SEQ ID NO: 15652 - protein, 9 aa, synthetic construct
GGNGFDTLT

SEQ ID NO: 15653 - protein, 9 aa, synthetic construct
GGDGNDKYK

SEQ ID NO: 15654 - protein, 9 aa, synthetic construct
GGDGDDIIM

SEQ ID NO: 15655 - protein, 9 aa, synthetic construct
GGSGADIAI

SEQ ID NO: 15656 - protein, 9 aa, synthetic construct
GGSGADIFF

SEQ ID NO: 15657 - protein, 9 aa, synthetic construct
GGSGADIFL

SEQ ID NO: 15658 - protein, 9 aa, synthetic construct
GGTGNDDIR

SEQ ID NO: 15659 - protein, 9 aa, synthetic construct
GGTGNDDIN

SEQ ID NO: 15660 - protein, 9 aa, synthetic construct
GGEGNDQLA

SEQ ID NO: 15661 - protein, 9 aa, synthetic construct
GGDGNDRME

SEQ ID NO: 15662 - protein, 9 aa, synthetic construct
GGIGHDTIL

SEQ ID NO: 15663 - protein, 9 aa, synthetic construct
GGAGNDVMG

SEQ ID NO: 15664 - protein, 9 aa, synthetic construct
GGDGSDELI

SEQ ID NO: 15665 - protein, 9 aa, synthetic construct
GGTGNDCLL

SEQ ID NO: 15666 - protein, 9 aa, synthetic construct
GGTGNDCLE

SEQ ID NO: 15667 - protein, 9 aa, synthetic construct
GGFGDDMLF

SEQ ID NO: 15668 - protein, 9 aa, synthetic construct
GGAGFDSLY

SEQ ID NO: 15669 - protein, 9 aa, synthetic construct
GGDGQDSVY

SEQ ID NO: 15670 - protein, 9 aa, synthetic construct
GGTGNDAMS

SEQ ID NO: 15671 - protein, 9 aa, synthetic construct
GGEGKDKIF

SEQ ID NO: 15672 - protein, 9 aa, synthetic construct
GGEGADTFN

SEQ ID NO: 15673 - protein, 9 aa, synthetic construct
GGAGFDVLT

SEQ ID NO: 15674 - protein, 9 aa, synthetic construct
GGAGFDTIY

SEQ ID NO: 15675 - protein, 9 aa, synthetic construct
GGNGADSLM

SEQ ID NO: 15676 - protein, 9 aa, synthetic construct
GGSGADLLL

SEQ ID NO: 15677 - protein, 9 aa, synthetic construct
GGTGLDTAS

SEQ ID NO: 15678 - protein, 9 aa, synthetic construct
GGAGFDTYV

SEQ ID NO: 15679 - protein, 9 aa, synthetic construct
GGDGNDLIH

SEQ ID NO: 15680 - protein, 9 aa, synthetic construct
GGEGNDNMS

SEQ ID NO: 15681 - protein, 9 aa, synthetic construct
GGTGLDSID

SEQ ID NO: 15682 - protein, 9 aa, synthetic construct
GGNGADSLW

SEQ ID NO: 15683 - protein, 9 aa, synthetic construct
GGTGADRLG

SEQ ID NO: 15684 - protein, 9 aa, synthetic construct
GGAGFDVIE

SEQ ID NO: 15685 - protein, 9 aa, synthetic construct
GGSGADLMV

SEQ ID NO: 15686 - protein, 9 aa, synthetic construct
GGLGTDELQ

SEQ ID NO: 15687 - protein, 9 aa, synthetic construct
GGKGRDWLE

SEQ ID NO: 15688 - protein, 9 aa, synthetic construct
GGTGADRLH

SEQ ID NO: 15689 - protein, 9 aa, synthetic construct
GGTGADRLL

SEQ ID NO: 15690 - protein, 9 aa, synthetic construct
GGSGADLYE

SEQ ID NO: 15691 - protein, 9 aa, synthetic construct
GGAGFDVLN

SEQ ID NO: 15692 - protein, 9 aa, synthetic construct
GGSGADMFG

SEQ ID NO: 15693 - protein, 9 aa, synthetic construct
GGFGTDDVF

SEQ ID NO: 15694 - protein, 9 aa, synthetic construct
GGAGFDTVS

SEQ ID NO: 15695 - protein, 9 aa, synthetic construct
GGNGDDVYV

SEQ ID NO: 15696 - protein, 9 aa, synthetic construct
GGSGADLLA

SEQ ID NO: 15697 - protein, 9 aa, synthetic construct
GGSGADLFI

SEQ ID NO: 15698 - protein, 9 aa, synthetic construct
GGIGIDAIW

SEQ ID NO: 15699 - protein, 9 aa, synthetic construct
GGAGFDTLE

SEQ ID NO: 15700 - protein, 9 aa, synthetic construct
GGDGSDAYY

SEQ ID NO: 15701 - protein, 9 aa, synthetic construct
GGNGADSLD

SEQ ID NO: 15702 - protein, 9 aa, synthetic construct
GGFGNDYLY

SEQ ID NO: 15703 - protein, 9 aa, synthetic construct
GGNGDDVYT

SEQ ID NO: 15704 - protein, 9 aa, synthetic construct
GGAGNDHFD

SEQ ID NO: 15705 - protein, 9 aa, synthetic construct
GGDGSDALL

SEQ ID NO: 15706 - protein, 9 aa, synthetic construct
GGDGNDLIA

SEQ ID NO: 15707 - protein, 9 aa, synthetic construct
GGLGSDTFL

SEQ ID NO: 15708 - protein, 9 aa, synthetic construct
GGTGLDTYR

SEQ ID NO: 15709 - protein, 9 aa, synthetic construct
GGTGLDTVS

SEQ ID NO: 15710 - protein, 9 aa, synthetic construct
GGDGSDALH

SEQ ID NO: 15711 - protein, 9 aa, synthetic construct
GGTGLDTMD

SEQ ID NO: 15712 - protein, 9 aa, synthetic construct
GGIGIDRMG

SEQ ID NO: 15713 - protein, 9 aa, synthetic construct
GGTGLDTLN

SEQ ID NO: 15714 - protein, 9 aa, synthetic construct
GGEGVDVLG

SEQ ID NO: 15715 - protein, 9 aa, synthetic construct
GGSGADLIW

SEQ ID NO: 15716 - protein, 9 aa, synthetic construct
GGTGNDLIW

SEQ ID NO: 15717 - protein, 9 aa, synthetic construct
GGTGADNFL

SEQ ID NO: 15718 - protein, 9 aa, synthetic construct
GGAGGDFFQ

SEQ ID NO: 15719 - protein, 9 aa, synthetic construct
GGTGADKVI

SEQ ID NO: 15720 - protein, 9 aa, synthetic construct
GGAGEDTVS

SEQ ID NO: 15721 - protein, 9 aa, synthetic construct
GGTGADLFL

SEQ ID NO: 15722 - protein, 9 aa, synthetic construct
GGRGNDTIQ

SEQ ID NO: 15723 - protein, 9 aa, synthetic construct
GGTGNDTVI

SEQ ID NO: 15724 - protein, 9 aa, synthetic construct
GGAGQDRFY

SEQ ID NO: 15725 - protein, 9 aa, synthetic construct
GGTGNDTVH

SEQ ID NO: 15726 - protein, 9 aa, synthetic construct
GGTGNDTVG

SEQ ID NO: 15727 - protein, 9 aa, synthetic construct
GGAGQDRFI

SEQ ID NO: 15728 - protein, 9 aa, synthetic construct
GGTGNDTMQ

SEQ ID NO: 15729 - protein, 9 aa, synthetic construct
GGIGDDTMD

SEQ ID NO: 15730 - protein, 9 aa, synthetic construct
GGAGEDTYV

SEQ ID NO: 15731 - protein, 9 aa, synthetic construct
GGRGNDTLG

SEQ ID NO: 15732 - protein, 9 aa, synthetic construct
GGTGNDTIR

SEQ ID NO: 15733 - protein, 9 aa, synthetic construct
GGDGNDSII

SEQ ID NO: 15734 - protein, 9 aa, synthetic construct
GGAGNDEVN

SEQ ID NO: 15735 - protein, 9 aa, synthetic construct
GGDGFDNLN

SEQ ID NO: 15736 - protein, 9 aa, synthetic construct
GGTGNDTFR

SEQ ID NO: 15737 - protein, 9 aa, synthetic construct
GGFGNDVLH

SEQ ID NO: 15738 - protein, 9 aa, synthetic construct
GGLGADKLW

SEQ ID NO: 15739 - protein, 9 aa, synthetic construct
GGLGADKMQ

SEQ ID NO: 15740 - protein, 9 aa, synthetic construct
GGTGNDTVT

SEQ ID NO: 15741 - protein, 9 aa, synthetic construct
GGEGHDLMS

SEQ ID NO: 15742 - protein, 9 aa, synthetic construct
GGAGEDTVL

SEQ ID NO: 15743 - protein, 9 aa, synthetic construct
GGAGIDILV

SEQ ID NO: 15744 - protein, 9 aa, synthetic construct
GGLGADLLF

SEQ ID NO: 15745 - protein, 9 aa, synthetic construct
GGEGHDLVD

SEQ ID NO: 15746 - protein, 9 aa, synthetic construct
GGIGDDTLH

SEQ ID NO: 15747 - protein, 9 aa, synthetic construct
GGFGDDSFH

SEQ ID NO: 15748 - protein, 9 aa, synthetic construct
GGRGNDSLE

SEQ ID NO: 15749 - protein, 9 aa, synthetic construct
GGGGADGFV

SEQ ID NO: 15750 - protein, 9 aa, synthetic construct
GGGGNDKLR

SEQ ID NO: 15751 - protein, 9 aa, synthetic construct
GGRGNDSLM

SEQ ID NO: 15752 - protein, 9 aa, synthetic construct
GGTGNDVIH

SEQ ID NO: 15753 - protein, 9 aa, synthetic construct
GGRGNDSLR

SEQ ID NO: 15754 - protein, 9 aa, synthetic construct
GGAGEDTLY

SEQ ID NO: 15755 - protein, 9 aa, synthetic construct
GGFGNDVLF

SEQ ID NO: 15756 - protein, 9 aa, synthetic construct
GGTGADKMS

SEQ ID NO: 15757 - protein, 9 aa, synthetic construct
GGTGNDVFL

SEQ ID NO: 15758 - protein, 9 aa, synthetic construct
GGRGNDTAQ

SEQ ID NO: 15759 - protein, 9 aa, synthetic construct
GGLGADKMV

SEQ ID NO: 15760 - protein, 9 aa, synthetic construct
GGTGNDTYA

SEQ ID NO: 15761 - protein, 9 aa, synthetic construct
GGRGNDTIA

SEQ ID NO: 15762 - protein, 9 aa, synthetic construct
GGSGKDRIE

SEQ ID NO: 15763 - protein, 9 aa, synthetic construct
GGRGNDTMW

SEQ ID NO: 15764 - protein, 9 aa, synthetic construct
GGTGNDTAY

SEQ ID NO: 15765 - protein, 9 aa, synthetic construct
GGAGQDQMN

SEQ ID NO: 15766 - protein, 9 aa, synthetic construct
GGAGEDVLH

SEQ ID NO: 15767 - protein, 9 aa, synthetic construct
GGTGADLIC

SEQ ID NO: 15768 - protein, 9 aa, synthetic construct
GGRGNDVMG

SEQ ID NO: 15769 - protein, 9 aa, synthetic construct
GGTGNDSMS

SEQ ID NO: 15770 - protein, 9 aa, synthetic construct
GGLGADIMS

SEQ ID NO: 15771 - protein, 9 aa, synthetic construct
GGKGKDLLV

SEQ ID NO: 15772 - protein, 9 aa, synthetic construct
GGRGNDVMT

SEQ ID NO: 15773 - protein, 9 aa, synthetic construct
GGLGADIMQ

SEQ ID NO: 15774 - protein, 9 aa, synthetic construct
GGKGKDLMI

SEQ ID NO: 15775 - protein, 9 aa, synthetic construct
GGEGTDTVS

SEQ ID NO: 15776 - protein, 9 aa, synthetic construct
GGRGNDVVT

SEQ ID NO: 15777 - protein, 9 aa, synthetic construct
GGLGADIMN

SEQ ID NO: 15778 - protein, 9 aa, synthetic construct
GGRGNDVYI

SEQ ID NO: 15779 - protein, 9 aa, synthetic construct
GGIGDDTYF

SEQ ID NO: 15780 - protein, 9 aa, synthetic construct
GGRGNDVYV

SEQ ID NO: 15781 - protein, 9 aa, synthetic construct
GGTGNDSMI

SEQ ID NO: 15782 - protein, 9 aa, synthetic construct
GGSGKDNLS

SEQ ID NO: 15783 - protein, 9 aa, synthetic construct
GGAGNDFAS

SEQ ID NO: 15784 - protein, 9 aa, synthetic construct
GGDGNDSFT

SEQ ID NO: 15785 - protein, 9 aa, synthetic construct
GGTGNDSVK

SEQ ID NO: 15786 - protein, 9 aa, synthetic construct
GGSGKDQLF

SEQ ID NO: 15787 - protein, 9 aa, synthetic construct
GGDGGDQFM

SEQ ID NO: 15788 - protein, 9 aa, synthetic construct
GGLGADKLD

SEQ ID NO: 15789 - protein, 9 aa, synthetic construct
GGAGNDEVT

SEQ ID NO: 15790 - protein, 9 aa, synthetic construct
GGDGSDLLH

SEQ ID NO: 15791 - protein, 9 aa, synthetic construct
GGAGQDQLT

SEQ ID NO: 15792 - protein, 9 aa, synthetic construct
GGSGKDQLT

SEQ ID NO: 15793 - protein, 9 aa, synthetic construct
GGRGNDTYS

SEQ ID NO: 15794 - protein, 9 aa, synthetic construct
GGIGDDTVD

SEQ ID NO: 15795 - protein, 9 aa, synthetic construct
GGRGNDVAF

SEQ ID NO: 15796 - protein, 9 aa, synthetic construct
GGDGNDFVV

SEQ ID NO: 15797 - protein, 9 aa, synthetic construct
GGEGDDSMS

SEQ ID NO: 15798 - protein, 9 aa, synthetic construct
GGAGEDVLD

SEQ ID NO: 15799 - protein, 9 aa, synthetic construct
GGTGNDSYH

SEQ ID NO: 15800 - protein, 9 aa, synthetic construct
GGIGDDTVL

SEQ ID NO: 15801 - protein, 9 aa, synthetic construct
GGTGNDSYA

SEQ ID NO: 15802 - protein, 9 aa, synthetic construct
GGRGNDVIF

SEQ ID NO: 15803 - protein, 9 aa, synthetic construct
GGNGHDALY

SEQ ID NO: 15804 - protein, 9 aa, synthetic construct
GGDGNDFYY

SEQ ID NO: 15805 - protein, 9 aa, synthetic construct
GGRGNDVLA

SEQ ID NO: 15806 - protein, 9 aa, synthetic construct
GGAGEDVLA

SEQ ID NO: 15807 - protein, 9 aa, synthetic construct
GGAGQDRMW

SEQ ID NO: 15808 - protein, 9 aa, synthetic construct
GGRGNDRVY

SEQ ID NO: 15809 - protein, 9 aa, synthetic construct
GGKGTDTLD

SEQ ID NO: 15810 - protein, 9 aa, synthetic construct
GGRGNDIYR

SEQ ID NO: 15811 - protein, 9 aa, synthetic construct
GGNGHDLLD

SEQ ID NO: 15812 - protein, 9 aa, synthetic construct
GGRGNDKIY

SEQ ID NO: 15813 - protein, 9 aa, synthetic construct
GGRGNDKLD

SEQ ID NO: 15814 - protein, 9 aa, synthetic construct
GGSGKDVFN

SEQ ID NO: 15815 - protein, 9 aa, synthetic construct
GGDGSDLYV

SEQ ID NO: 15816 - protein, 9 aa, synthetic construct
GGRGNDKLN

SEQ ID NO: 15817 - protein, 9 aa, synthetic construct
GGEGTDTAA

SEQ ID NO: 15818 - protein, 9 aa, synthetic construct
GGDGNDFLI

SEQ ID NO: 15819 - protein, 9 aa, synthetic construct
GGTGNDYMV

SEQ ID NO: 15820 - protein, 9 aa, synthetic construct
GGTGNDYMR

SEQ ID NO: 15821 - protein, 9 aa, synthetic construct
GGRGNDLIL

SEQ ID NO: 15822 - protein, 9 aa, synthetic construct
GGLGADNLI

SEQ ID NO: 15823 - protein, 9 aa, synthetic construct
GGEGDDLVR

SEQ ID NO: 15824 - protein, 9 aa, synthetic construct
GGRGNDLLF

SEQ ID NO: 15825 - protein, 9 aa, synthetic construct
GGFGDDSIQ

SEQ ID NO: 15826 - protein, 9 aa, synthetic construct
GGSGKDTMN

SEQ ID NO: 15827 - protein, 9 aa, synthetic construct
GGAGNDELQ

SEQ ID NO: 15828 - protein, 9 aa, synthetic construct
GGDGNDFLL

SEQ ID NO: 15829 - protein, 9 aa, synthetic construct
GGLGADNLD

SEQ ID NO: 15830 - protein, 9 aa, synthetic construct
GGIGDDSLF

SEQ ID NO: 15831 - protein, 9 aa, synthetic construct
GGIGDDSLA

SEQ ID NO: 15832 - protein, 9 aa, synthetic construct
GGTGNDVLG

SEQ ID NO: 15833 - protein, 9 aa, synthetic construct
GGDGNDFIY

SEQ ID NO: 15834 - protein, 9 aa, synthetic construct
GGTGADILH

SEQ ID NO: 15835 - protein, 9 aa, synthetic construct
GGRGNDHVG

SEQ ID NO: 15836 - protein, 9 aa, synthetic construct
GGAGQDTMS

SEQ ID NO: 15837 - protein, 9 aa, synthetic construct
GGLGADQLI

SEQ ID NO: 15838 - protein, 9 aa, synthetic construct
GGRGNDIIA

SEQ ID NO: 15839 - protein, 9 aa, synthetic construct
GGAGQDTMI

SEQ ID NO: 15840 - protein, 9 aa, synthetic construct
GGNGHDLLF

SEQ ID NO: 15841 - protein, 9 aa, synthetic construct
GGAGQDTLY

SEQ ID NO: 15842 - protein, 9 aa, synthetic construct
GGIGDDRYR

SEQ ID NO: 15843 - protein, 9 aa, synthetic construct
GGTGADILL

SEQ ID NO: 15844 - protein, 9 aa, synthetic construct
GGEGNDRYT

SEQ ID NO: 15845 - protein, 9 aa, synthetic construct
GGTGQDALN

SEQ ID NO: 15846 - protein, 9 aa, synthetic construct
GGAGNDELK

SEQ ID NO: 15847 - protein, 9 aa, synthetic construct
GGEGNDRYF

SEQ ID NO: 15848 - protein, 9 aa, synthetic construct
GGSGKDVIV

SEQ ID NO: 15849 - protein, 9 aa, synthetic construct
GGRGNDILN

SEQ ID NO: 15850 - protein, 9 aa, synthetic construct
GGEGTDSLF

SEQ ID NO: 15851 - protein, 9 aa, synthetic construct
GGLGRDTID

SEQ ID NO: 15852 - protein, 9 aa, synthetic construct
GGAGEDSIL

SEQ ID NO: 15853 - protein, 9 aa, synthetic construct
GGTGNDYLL

SEQ ID NO: 15854 - protein, 9 aa, synthetic construct
GGDGSDLVS

SEQ ID NO: 15855 - protein, 9 aa, synthetic construct
GGRGNDLLV

SEQ ID NO: 15856 - protein, 9 aa, synthetic construct
GGLGADNIG

SEQ ID NO: 15857 - protein, 9 aa, synthetic construct
GGLGADLMQ

SEQ ID NO: 15858 - protein, 9 aa, synthetic construct
GGDGDDSYV

SEQ ID NO: 15859 - protein, 9 aa, synthetic construct
GGTGNDWID

SEQ ID NO: 15860 - protein, 9 aa, synthetic construct
GGAGQDSLI

SEQ ID NO: 15861 - protein, 9 aa, synthetic construct
GGEGTDTIA

SEQ ID NO: 15862 - protein, 9 aa, synthetic construct
GGDGSDLLY

SEQ ID NO: 15863 - protein, 9 aa, synthetic construct
GGAGEDTIW

SEQ ID NO: 15864 - protein, 9 aa, synthetic construct
GGRGNDRLA

SEQ ID NO: 15865 - protein, 9 aa, synthetic construct
GGAGEDTLA

SEQ ID NO: 15866 - protein, 9 aa, synthetic construct
GGAGNDEME

SEQ ID NO: 15867 - protein, 9 aa, synthetic construct
GGTGNDVYF

SEQ ID NO: 15868 - protein, 9 aa, synthetic construct
GGRGNDRLK

SEQ ID NO: 15869 - protein, 9 aa, synthetic construct
GGRGNDRLQ

SEQ ID NO: 15870 - protein, 9 aa, synthetic construct
GGTGADKLW

SEQ ID NO: 15871 - protein, 9 aa, synthetic construct
GGAGNDEMF

SEQ ID NO: 15872 - protein, 9 aa, synthetic construct
GGTGNDVMK

SEQ ID NO: 15873 - protein, 9 aa, synthetic construct
GGAGNDEMH

SEQ ID NO: 15874 - protein, 9 aa, synthetic construct
GGTGNDVMD

SEQ ID NO: 15875 - protein, 9 aa, synthetic construct
GGRGNDRMY

SEQ ID NO: 15876 - protein, 9 aa, synthetic construct
GGRGNDQLS

SEQ ID NO: 15877 - protein, 9 aa, synthetic construct
GGGGNDTIR

SEQ ID NO: 15878 - protein, 9 aa, synthetic construct
GGAGQDSLV

SEQ ID NO: 15879 - protein, 9 aa, synthetic construct
GGDGSDLMR

SEQ ID NO: 15880 - protein, 9 aa, synthetic construct
GGRGNDLLY

SEQ ID NO: 15881 - protein, 9 aa, synthetic construct
GGGGHDSLD

SEQ ID NO: 15882 - protein, 9 aa, synthetic construct
GGGGNDKLE

SEQ ID NO: 15883 - protein, 9 aa, synthetic construct
GGLGTDSLD

SEQ ID NO: 15884 - protein, 9 aa, synthetic construct
GGLGADMLT

SEQ ID NO: 15885 - protein, 9 aa, synthetic construct
GGAGEDTFR

SEQ ID NO: 15886 - protein, 9 aa, synthetic construct
GGSGKDTLN

SEQ ID NO: 15887 - protein, 9 aa, synthetic construct
GGAGEDTID

SEQ ID NO: 15888 - protein, 9 aa, synthetic construct
GGLGRDTIV

SEQ ID NO: 15889 - protein, 9 aa, synthetic construct
GGEGHDLLD

SEQ ID NO: 15890 - protein, 9 aa, synthetic construct
GGTGNDWMN

SEQ ID NO: 15891 - protein, 9 aa, synthetic construct
GGTGADIVF

SEQ ID NO: 15892 - protein, 9 aa, synthetic construct
GGAGIDKLI

SEQ ID NO: 15893 - protein, 9 aa, synthetic construct
GGSGKDTLH

SEQ ID NO: 15894 - protein, 9 aa, synthetic construct
GGDGDDNLR

SEQ ID NO: 15895 - protein, 9 aa, synthetic construct
GGFGDDSIG

SEQ ID NO: 15896 - protein, 9 aa, synthetic construct
GGLGADLMV

SEQ ID NO: 15897 - protein, 9 aa, synthetic construct
GGNGDDIFV

SEQ ID NO: 15898 - protein, 9 aa, synthetic construct
GGAGQDNFV

SEQ ID NO: 15899 - protein, 9 aa, synthetic construct
GGEGNDFVK

SEQ ID NO: 15900 - protein, 9 aa, synthetic construct
GGRGNDYAH

SEQ ID NO: 15901 - protein, 9 aa, synthetic construct
GGAGFDDLY

SEQ ID NO: 15902 - protein, 9 aa, synthetic construct
GGDGNDIAW

SEQ ID NO: 15903 - protein, 9 aa, synthetic construct
GGRGRDVLD

SEQ ID NO: 15904 - protein, 9 aa, synthetic construct
GGKGWDRLV

SEQ ID NO: 15905 - protein, 9 aa, synthetic construct
GGRGRDVLH

SEQ ID NO: 15906 - protein, 9 aa, synthetic construct
GGEGHDTID

SEQ ID NO: 15907 - protein, 9 aa, synthetic construct
GGDGSDLFM

SEQ ID NO: 15908 - protein, 9 aa, synthetic construct
GGRGRDVLN

SEQ ID NO: 15909 - protein, 9 aa, synthetic construct
GGAGQDAFV

SEQ ID NO: 15910 - protein, 9 aa, synthetic construct
GGEGNDRIW

SEQ ID NO: 15911 - protein, 9 aa, synthetic construct
GGDGDDHLT

SEQ ID NO: 15912 - protein, 9 aa, synthetic construct
GGAGFDELT

SEQ ID NO: 15913 - protein, 9 aa, synthetic construct
GGGGNDLLG

SEQ ID NO: 15914 - protein, 9 aa, synthetic construct
GGNGGDNFL

SEQ ID NO: 15915 - protein, 9 aa, synthetic construct
GGGGADAFV

SEQ ID NO: 15916 - protein, 9 aa, synthetic construct
GGAGFDFAL

SEQ ID NO: 15917 - protein, 9 aa, synthetic construct
GGSGKDIFL

SEQ ID NO: 15918 - protein, 9 aa, synthetic construct
GGAGIDIAA

SEQ ID NO: 15919 - protein, 9 aa, synthetic construct
GGTGADMLN

SEQ ID NO: 15920 - protein, 9 aa, synthetic construct
GGEGHDTLE

SEQ ID NO: 15921 - protein, 9 aa, synthetic construct
GGRGRDVFV

SEQ ID NO: 15922 - protein, 9 aa, synthetic construct
GGGGADALD

SEQ ID NO: 15923 - protein, 9 aa, synthetic construct
GGTGNDSLG

SEQ ID NO: 15924 - protein, 9 aa, synthetic construct
GGTGNDNMN

SEQ ID NO: 15925 - protein, 9 aa, synthetic construct
GGTGNDQIT

SEQ ID NO: 15926 - protein, 9 aa, synthetic construct
GGGGNDLIV

SEQ ID NO: 15927 - protein, 9 aa, synthetic construct
GGGGADALK

SEQ ID NO: 15928 - protein, 9 aa, synthetic construct
GGTGNDQIS

SEQ ID NO: 15929 - protein, 9 aa, synthetic construct
GGKGYDTLR

SEQ ID NO: 15930 - protein, 9 aa, synthetic construct
GGRGRDTIL

SEQ ID NO: 15931 - protein, 9 aa, synthetic construct
GGTGADMIY

SEQ ID NO: 15932 - protein, 9 aa, synthetic construct
GGRGRDTIT

SEQ ID NO: 15933 - protein, 9 aa, synthetic construct
GGDGFDQIR

SEQ ID NO: 15934 - protein, 9 aa, synthetic construct
GGDGDDHLE

SEQ ID NO: 15935 - protein, 9 aa, synthetic construct
GGRGRDTLE

SEQ ID NO: 15936 - protein, 9 aa, synthetic construct
GGNGADNIL

SEQ ID NO: 15937 - protein, 9 aa, synthetic construct
GGAGFDDLD

SEQ ID NO: 15938 - protein, 9 aa, synthetic construct
GGNGGDRLE

SEQ ID NO: 15939 - protein, 9 aa, synthetic construct
GGDGFDQLD

SEQ ID NO: 15940 - protein, 9 aa, synthetic construct
GGDGNDIAS

SEQ ID NO: 15941 - protein, 9 aa, synthetic construct
GGAGQDALY

SEQ ID NO: 15942 - protein, 9 aa, synthetic construct
GGAGQDALV

SEQ ID NO: 15943 - protein, 9 aa, synthetic construct
GGRGRDTVH

SEQ ID NO: 15944 - protein, 9 aa, synthetic construct
GGRGSDELQ

SEQ ID NO: 15945 - protein, 9 aa, synthetic construct
GGEGDDTFY

SEQ ID NO: 15946 - protein, 9 aa, synthetic construct
GGEGHDTLI

SEQ ID NO: 15947 - protein, 9 aa, synthetic construct
GGFGDDRLE

SEQ ID NO: 15948 - protein, 9 aa, synthetic construct
GGIGEDILI

SEQ ID NO: 15949 - protein, 9 aa, synthetic construct
GGTGNDLVL

SEQ ID NO: 15950 - protein, 9 aa, synthetic construct
GGRGSDLMQ

SEQ ID NO: 15951 - protein, 9 aa, synthetic construct
GGAGPDRLR

SEQ ID NO: 15952 - protein, 9 aa, synthetic construct
GGKGTDVLD

SEQ ID NO: 15953 - protein, 9 aa, synthetic construct
GGAGNDFLM

SEQ ID NO: 15954 - protein, 9 aa, synthetic construct
GGTGNDLMY

SEQ ID NO: 15955 - protein, 9 aa, synthetic construct
GGKGTDVFI

SEQ ID NO: 15956 - protein, 9 aa, synthetic construct
GGAGIDHLS

SEQ ID NO: 15957 - protein, 9 aa, synthetic construct
GGAGIDHLR

SEQ ID NO: 15958 - protein, 9 aa, synthetic construct
GGGGNDQLA

SEQ ID NO: 15959 - protein, 9 aa, synthetic construct
GGAGPDRLA

SEQ ID NO: 15960 - protein, 9 aa, synthetic construct
GGEGHDTLT

SEQ ID NO: 15961 - protein, 9 aa, synthetic construct
GGEGHDTLV

SEQ ID NO: 15962 - protein, 9 aa, synthetic construct
GGDGNDRYT

SEQ ID NO: 15963 - protein, 9 aa, synthetic construct
GGLGRDVVA

SEQ ID NO: 15964 - protein, 9 aa, synthetic construct
GGIGEDTAL

SEQ ID NO: 15965 - protein, 9 aa, synthetic construct
GGAGPDQLT

SEQ ID NO: 15966 - protein, 9 aa, synthetic construct
GGTGADNFD

SEQ ID NO: 15967 - protein, 9 aa, synthetic construct
GGTGNDLVR

SEQ ID NO: 15968 - protein, 9 aa, synthetic construct
GGAGFDIAD

SEQ ID NO: 15969 - protein, 9 aa, synthetic construct
GGTGNDLVW

SEQ ID NO: 15970 - protein, 9 aa, synthetic construct
GGLGRDVMS

SEQ ID NO: 15971 - protein, 9 aa, synthetic construct
GGEGDDTVL

SEQ ID NO: 15972 - protein, 9 aa, synthetic construct
GGEGNDRIS

SEQ ID NO: 15973 - protein, 9 aa, synthetic construct
GGAGPDTLT

SEQ ID NO: 15974 - protein, 9 aa, synthetic construct
GGAGPDTLS

SEQ ID NO: 15975 - protein, 9 aa, synthetic construct
GGAGFDFLV

SEQ ID NO: 15976 - protein, 9 aa, synthetic construct
GGAGFDGAD

SEQ ID NO: 15977 - protein, 9 aa, synthetic construct
GGRGSDILN

SEQ ID NO: 15978 - protein, 9 aa, synthetic construct
GGKGKDRLW

SEQ ID NO: 15979 - protein, 9 aa, synthetic construct
GGAGPDTLA

SEQ ID NO: 15980 - protein, 9 aa, synthetic construct
GGTGNDLYI

SEQ ID NO: 15981 - protein, 9 aa, synthetic construct
GGDGNDIIH

SEQ ID NO: 15982 - protein, 9 aa, synthetic construct
GGRGSDIYR

SEQ ID NO: 15983 - protein, 9 aa, synthetic construct
GGRGSDKLL

SEQ ID NO: 15984 - protein, 9 aa, synthetic construct
GGDGSDKLS

SEQ ID NO: 15985 - protein, 9 aa, synthetic construct
GGKGVDILT

SEQ ID NO: 15986 - protein, 9 aa, synthetic construct
GGTGNDMID

SEQ ID NO: 15987 - protein, 9 aa, synthetic construct
GGAGFDHMF

SEQ ID NO: 15988 - protein, 9 aa, synthetic construct
GGTGNDLYR

SEQ ID NO: 15989 - protein, 9 aa, synthetic construct
GGTGADLMT

SEQ ID NO: 15990 - protein, 9 aa, synthetic construct
GGTGADLMS

SEQ ID NO: 15991 - protein, 9 aa, synthetic construct
GGTGNDQLE

SEQ ID NO: 15992 - protein, 9 aa, synthetic construct
GGAGQDKLT

SEQ ID NO: 15993 - protein, 9 aa, synthetic construct
GGDGNDGLQ

SEQ ID NO: 15994 - protein, 9 aa, synthetic construct
GGRGQDLLD

SEQ ID NO: 15995 - protein, 9 aa, synthetic construct
GGIGDDVFI

SEQ ID NO: 15996 - protein, 9 aa, synthetic construct
GGDGSDLLE

SEQ ID NO: 15997 - protein, 9 aa, synthetic construct
GGSGKDLLN

SEQ ID NO: 15998 - protein, 9 aa, synthetic construct
GGDGGDPLD

SEQ ID NO: 15999 - protein, 9 aa, synthetic construct
GGDGFDTLA

SEQ ID NO: 16000 - protein, 9 aa, synthetic construct
GGSGKDLLK

SEQ ID NO: 16001 - protein, 9 aa, synthetic construct
GGLGADFMR

SEQ ID NO: 16002 - protein, 9 aa, synthetic construct
GGSGKDLLI

SEQ ID NO: 16003 - protein, 9 aa, synthetic construct
GGEGTDVLS

SEQ ID NO: 16004 - protein, 9 aa, synthetic construct
GGDGDDGMQ

SEQ ID NO: 16005 - protein, 9 aa, synthetic construct
GGEGNDFVL

SEQ ID NO: 16006 - protein, 9 aa, synthetic construct
GGGGNDQLG

SEQ ID NO: 16007 - protein, 9 aa, synthetic construct
GGGGADDLV

SEQ ID NO: 16008 - protein, 9 aa, synthetic construct
GGGGADDLT

SEQ ID NO: 16009 - protein, 9 aa, synthetic construct
GGTGNDRMI

SEQ ID NO: 16010 - protein, 9 aa, synthetic construct
GGDGSDLLA

SEQ ID NO: 16011 - protein, 9 aa, synthetic construct
GGAGNDFFY

SEQ ID NO: 16012 - protein, 9 aa, synthetic construct
GGAGQDLLM

SEQ ID NO: 16013 - protein, 9 aa, synthetic construct
GGDGNDGLN

SEQ ID NO: 16014 - protein, 9 aa, synthetic construct
GGLGRDTMG

SEQ ID NO: 16015 - protein, 9 aa, synthetic construct
GGGGGDSLI

SEQ ID NO: 16016 - protein, 9 aa, synthetic construct
GGDGNDGIG

SEQ ID NO: 16017 - protein, 9 aa, synthetic construct
GGRGNDYLL

SEQ ID NO: 16018 - protein, 9 aa, synthetic construct
GGDGDDGLF

SEQ ID NO: 16019 - protein, 9 aa, synthetic construct
GGIGDDTYI

SEQ ID NO: 16020 - protein, 9 aa, synthetic construct
GGIGDDTYL

SEQ ID NO: 16021 - protein, 9 aa, synthetic construct
GGTGADLLE

SEQ ID NO: 16022 - protein, 9 aa, synthetic construct
GGRGNDYVK

SEQ ID NO: 16023 - protein, 9 aa, synthetic construct
GGTGNDSIK

SEQ ID NO: 16024 - protein, 9 aa, synthetic construct
GGDGDDGLN

SEQ ID NO: 16025 - protein, 9 aa, synthetic construct
GGAGQDLLS

SEQ ID NO: 16026 - protein, 9 aa, synthetic construct
GGTGNDSIF

SEQ ID NO: 16027 - protein, 9 aa, synthetic construct
GGTGNDSIE

SEQ ID NO: 16028 - protein, 9 aa, synthetic construct
GGIGDDTYY

SEQ ID NO: 16029 - protein, 9 aa, synthetic construct
GGAGEDVMF

SEQ ID NO: 16030 - protein, 9 aa, synthetic construct
GGGGNDQLL

SEQ ID NO: 16031 - protein, 9 aa, synthetic construct
GGDGNDGLD

SEQ ID NO: 16032 - protein, 9 aa, synthetic construct
GGRGQDFIF

SEQ ID NO: 16033 - protein, 9 aa, synthetic construct
GGAGQDLLT

SEQ ID NO: 16034 - protein, 9 aa, synthetic construct
GGLGADELR

SEQ ID NO: 16035 - protein, 9 aa, synthetic construct
GGTGNDRLQ

SEQ ID NO: 16036 - protein, 9 aa, synthetic construct
GGTGNDQLH

SEQ ID NO: 16037 - protein, 9 aa, synthetic construct
GGTGNDRLK

SEQ ID NO: 16038 - protein, 9 aa, synthetic construct
GGTGNDQVE

SEQ ID NO: 16039 - protein, 9 aa, synthetic construct
GGIGSDVLN

SEQ ID NO: 16040 - protein, 9 aa, synthetic construct
GGLGADALS

SEQ ID NO: 16041 - protein, 9 aa, synthetic construct
GGTGNDQMS

SEQ ID NO: 16042 - protein, 9 aa, synthetic construct
GGGGADAMT

SEQ ID NO: 16043 - protein, 9 aa, synthetic construct
GGAGQDFLI

SEQ ID NO: 16044 - protein, 9 aa, synthetic construct
GGGGNDLIM

SEQ ID NO: 16045 - protein, 9 aa, synthetic construct
GGTGNDQMK

SEQ ID NO: 16046 - protein, 9 aa, synthetic construct
GGNGGDTFV

SEQ ID NO: 16047 - protein, 9 aa, synthetic construct
GGSGKDKFV

SEQ ID NO: 16048 - protein, 9 aa, synthetic construct
GGAGNDFII

SEQ ID NO: 16049 - protein, 9 aa, synthetic construct
GGTGNDQMA

SEQ ID NO: 16050 - protein, 9 aa, synthetic construct
GGRGRDRLE

SEQ ID NO: 16051 - protein, 9 aa, synthetic construct
GGLGRDVLK

SEQ ID NO: 16052 - protein, 9 aa, synthetic construct
GGAGQDEMT

SEQ ID NO: 16053 - protein, 9 aa, synthetic construct
GGDGNDSAL

SEQ ID NO: 16054 - protein, 9 aa, synthetic construct
GGGGNDLIQ

SEQ ID NO: 16055 - protein, 9 aa, synthetic construct
GGRGRDRMY

SEQ ID NO: 16056 - protein, 9 aa, synthetic construct
GGSGKDILY

SEQ ID NO: 16057 - protein, 9 aa, synthetic construct
GGRGRDLMT

SEQ ID NO: 16058 - protein, 9 aa, synthetic construct
GGDGSDLIR

SEQ ID NO: 16059 - protein, 9 aa, synthetic construct
GGRGRDLLQ

SEQ ID NO: 16060 - protein, 9 aa, synthetic construct
GGSGKDKLY

SEQ ID NO: 16061 - protein, 9 aa, synthetic construct
GGDGDDGVY

SEQ ID NO: 16062 - protein, 9 aa, synthetic construct
GGNGGDTLR

SEQ ID NO: 16063 - protein, 9 aa, synthetic construct
GGIGDDVID

SEQ ID NO: 16064 - protein, 9 aa, synthetic construct
GGRGRDDLS

SEQ ID NO: 16065 - protein, 9 aa, synthetic construct
GGSGKDKMS

SEQ ID NO: 16066 - protein, 9 aa, synthetic construct
GGLGRDVFR

SEQ ID NO: 16067 - protein, 9 aa, synthetic construct
GGIGDDVII

SEQ ID NO: 16068 - protein, 9 aa, synthetic construct
GGEGNDRLQ

SEQ ID NO: 16069 - protein, 9 aa, synthetic construct
GGRGRDHLF

SEQ ID NO: 16070 - protein, 9 aa, synthetic construct
GGTGNDRFI

SEQ ID NO: 16071 - protein, 9 aa, synthetic construct
GGAGEDWLD

SEQ ID NO: 16072 - protein, 9 aa, synthetic construct
GGDGNDHLE

SEQ ID NO: 16073 - protein, 9 aa, synthetic construct
GGDGNDHLF

SEQ ID NO: 16074 - protein, 9 aa, synthetic construct
GGTGADLLY

SEQ ID NO: 16075 - protein, 9 aa, synthetic construct
GGSGKDKLH

SEQ ID NO: 16076 - protein, 9 aa, synthetic construct
GGIGDDVIV

SEQ ID NO: 16077 - protein, 9 aa, synthetic construct
GGAGQDIIH

SEQ ID NO: 16078 - protein, 9 aa, synthetic construct
GGSGKDKLF

SEQ ID NO: 16079 - protein, 9 aa, synthetic construct
GGEGNDMLL

SEQ ID NO: 16080 - protein, 9 aa, synthetic construct
GGSGADSME

SEQ ID NO: 16081 - protein, 9 aa, synthetic construct
GGIGDDRYI

SEQ ID NO: 16082 - protein, 9 aa, synthetic construct
GGSGDDTMS

SEQ ID NO: 16083 - protein, 9 aa, synthetic construct
GGTGDDVAA

SEQ ID NO: 16084 - protein, 9 aa, synthetic construct
GGTGDDTYW

SEQ ID NO: 16085 - protein, 9 aa, synthetic construct
GGIGNDTYT

SEQ ID NO: 16086 - protein, 9 aa, synthetic construct
GGAGHDIYL

SEQ ID NO: 16087 - protein, 9 aa, synthetic construct
GGSGDDTVN

SEQ ID NO: 16088 - protein, 9 aa, synthetic construct
GGTGDDTVE

SEQ ID NO: 16089 - protein, 9 aa, synthetic construct
GGTGDDTMV

SEQ ID NO: 16090 - protein, 9 aa, synthetic construct
GGGGNDTYF

SEQ ID NO: 16091 - protein, 9 aa, synthetic construct
GGSGDDTYR

SEQ ID NO: 16092 - protein, 9 aa, synthetic construct
GGGGGDILN

SEQ ID NO: 16093 - protein, 9 aa, synthetic construct
GGIGNDVFI

SEQ ID NO: 16094 - protein, 9 aa, synthetic construct
GGTGDDTML

SEQ ID NO: 16095 - protein, 9 aa, synthetic construct
GGKGNDTLF

SEQ ID NO: 16096 - protein, 9 aa, synthetic construct
GGTGDDTIW

SEQ ID NO: 16097 - protein, 9 aa, synthetic construct
GGTGDDTIR

SEQ ID NO: 16098 - protein, 9 aa, synthetic construct
GGTGDDTIM

SEQ ID NO: 16099 - protein, 9 aa, synthetic construct
GGTGDDDLF

SEQ ID NO: 16100 - protein, 9 aa, synthetic construct
GGSGGDTIT

SEQ ID NO: 16101 - protein, 9 aa, synthetic construct
GGSGGDTIR

SEQ ID NO: 16102 - protein, 9 aa, synthetic construct
GGTGDDVAH

SEQ ID NO: 16103 - protein, 9 aa, synthetic construct
GGAGHDIYF

SEQ ID NO: 16104 - protein, 9 aa, synthetic construct
GGTGDDVYY

SEQ ID NO: 16105 - protein, 9 aa, synthetic construct
GGEGADWID

SEQ ID NO: 16106 - protein, 9 aa, synthetic construct
GGDGDDIYR

SEQ ID NO: 16107 - protein, 9 aa, synthetic construct
GGSGDDTIH

SEQ ID NO: 16108 - protein, 9 aa, synthetic construct
GGSGDDTIR

SEQ ID NO: 16109 - protein, 9 aa, synthetic construct
GGDGRDLLN

SEQ ID NO: 16110 - protein, 9 aa, synthetic construct
GGIGNDTVL

SEQ ID NO: 16111 - protein, 9 aa, synthetic construct
GGTGDDVMS

SEQ ID NO: 16112 - protein, 9 aa, synthetic construct
GGIGNDTVT

SEQ ID NO: 16113 - protein, 9 aa, synthetic construct
GGTGDDALR

SEQ ID NO: 16114 - protein, 9 aa, synthetic construct
GGEGDDMLY

SEQ ID NO: 16115 - protein, 9 aa, synthetic construct
GGDGGDHMD

SEQ ID NO: 16116 - protein, 9 aa, synthetic construct
GGTGDDVLK

SEQ ID NO: 16117 - protein, 9 aa, synthetic construct
GGFGADTVV

SEQ ID NO: 16118 - protein, 9 aa, synthetic construct
GGTGDDVIV

SEQ ID NO: 16119 - protein, 9 aa, synthetic construct
GGAGNDKII

SEQ ID NO: 16120 - protein, 9 aa, synthetic construct
GGTGDDVIS

SEQ ID NO: 16121 - protein, 9 aa, synthetic construct
GGTGDDAYV

SEQ ID NO: 16122 - protein, 9 aa, synthetic construct
GGDGDDRAY

SEQ ID NO: 16123 - protein, 9 aa, synthetic construct
GGDGRDALY

SEQ ID NO: 16124 - protein, 9 aa, synthetic construct
GGTGDDVIA

SEQ ID NO: 16125 - protein, 9 aa, synthetic construct
GGGGNDTYG

SEQ ID NO: 16126 - protein, 9 aa, synthetic construct
GGTGDDDLN

SEQ ID NO: 16127 - protein, 9 aa, synthetic construct
GGSGDDVIK

SEQ ID NO: 16128 - protein, 9 aa, synthetic construct
GGIGNDVIN

SEQ ID NO: 16129 - protein, 9 aa, synthetic construct
GGAGNDQIN

SEQ ID NO: 16130 - protein, 9 aa, synthetic construct
GGAGNDQIL

SEQ ID NO: 16131 - protein, 9 aa, synthetic construct
GGNGEDSLY

SEQ ID NO: 16132 - protein, 9 aa, synthetic construct
GGTGDDSIW

SEQ ID NO: 16133 - protein, 9 aa, synthetic construct
GGSGDDVVR

SEQ ID NO: 16134 - protein, 9 aa, synthetic construct
GGTGDDEIT

SEQ ID NO: 16135 - protein, 9 aa, synthetic construct
GGAGHDLLA

SEQ ID NO: 16136 - protein, 9 aa, synthetic construct
GGNGEDSLF

SEQ ID NO: 16137 - protein, 9 aa, synthetic construct
GGSGDDWFN

SEQ ID NO: 16138 - protein, 9 aa, synthetic construct
GGTGDDSFI

SEQ ID NO: 16139 - protein, 9 aa, synthetic construct
GGGGGDILT

SEQ ID NO: 16140 - protein, 9 aa, synthetic construct
GGSGDDWIE

SEQ ID NO: 16141 - protein, 9 aa, synthetic construct
GGAGNDQFV

SEQ ID NO: 16142 - protein, 9 aa, synthetic construct
GGSGDDWLA

SEQ ID NO: 16143 - protein, 9 aa, synthetic construct
GGDGRDDIK

SEQ ID NO: 16144 - protein, 9 aa, synthetic construct
GGTGDDRYV

SEQ ID NO: 16145 - protein, 9 aa, synthetic construct
GGSGDDWLS

SEQ ID NO: 16146 - protein, 9 aa, synthetic construct
GGAGHDTIR

SEQ ID NO: 16147 - protein, 9 aa, synthetic construct
GGSGDDWML

SEQ ID NO: 16148 - protein, 9 aa, synthetic construct
GGTGDDSLG

SEQ ID NO: 16149 - protein, 9 aa, synthetic construct
GGSGDDVMT

SEQ ID NO: 16150 - protein, 9 aa, synthetic construct
GGAGHDLIV

SEQ ID NO: 16151 - protein, 9 aa, synthetic construct
GGAGHDLIE

SEQ ID NO: 16152 - protein, 9 aa, synthetic construct
GGTGDDTAV

SEQ ID NO: 16153 - protein, 9 aa, synthetic construct
GGIGNDVIV

SEQ ID NO: 16154 - protein, 9 aa, synthetic construct
GGIGNDVIY

SEQ ID NO: 16155 - protein, 9 aa, synthetic construct
GGSGGDTIA

SEQ ID NO: 16156 - protein, 9 aa, synthetic construct
GGTGDDSYW

SEQ ID NO: 16157 - protein, 9 aa, synthetic construct
GGEGNDIMK

SEQ ID NO: 16158 - protein, 9 aa, synthetic construct
GGTGDDDLS

SEQ ID NO: 16159 - protein, 9 aa, synthetic construct
GGTGDDSVT

SEQ ID NO: 16160 - protein, 9 aa, synthetic construct
GGTGDDDLY

SEQ ID NO: 16161 - protein, 9 aa, synthetic construct
GGFGDDILI

SEQ ID NO: 16162 - protein, 9 aa, synthetic construct
GGGGNDTYH

SEQ ID NO: 16163 - protein, 9 aa, synthetic construct
GGTGDDSMY

SEQ ID NO: 16164 - protein, 9 aa, synthetic construct
GGSGDDVLM

SEQ ID NO: 16165 - protein, 9 aa, synthetic construct
GGFGDDILQ

SEQ ID NO: 16166 - protein, 9 aa, synthetic construct
GGSGDDVLQ

SEQ ID NO: 16167 - protein, 9 aa, synthetic construct
GGNGDDYLA

SEQ ID NO: 16168 - protein, 9 aa, synthetic construct
GGTGDDSLQ

SEQ ID NO: 16169 - protein, 9 aa, synthetic construct
GGSGDDVMD

SEQ ID NO: 16170 - protein, 9 aa, synthetic construct
GGTGDDVYT

SEQ ID NO: 16171 - protein, 9 aa, synthetic construct
GGNGDDAFV

SEQ ID NO: 16172 - protein, 9 aa, synthetic construct
GGAGGDYLN

SEQ ID NO: 16173 - protein, 9 aa, synthetic construct
GGDGRDLVY

SEQ ID NO: 16174 - protein, 9 aa, synthetic construct
GGSGDDRLH

SEQ ID NO: 16175 - protein, 9 aa, synthetic construct
GGDGNDNIG

SEQ ID NO: 16176 - protein, 9 aa, synthetic construct
GGEGNDKLE

SEQ ID NO: 16177 - protein, 9 aa, synthetic construct
GGIGNDTAI

SEQ ID NO: 16178 - protein, 9 aa, synthetic construct
GGIGNDTFD

SEQ ID NO: 16179 - protein, 9 aa, synthetic construct
GGAGHDAVT

SEQ ID NO: 16180 - protein, 9 aa, synthetic construct
GGDGNDNIH

SEQ ID NO: 16181 - protein, 9 aa, synthetic construct
GGIGNDTFL

SEQ ID NO: 16182 - protein, 9 aa, synthetic construct
GGSGGDYLV

SEQ ID NO: 16183 - protein, 9 aa, synthetic construct
GGAGHDTYI

SEQ ID NO: 16184 - protein, 9 aa, synthetic construct
GGAGNDRFF

SEQ ID NO: 16185 - protein, 9 aa, synthetic construct
GGSGDDRMI

SEQ ID NO: 16186 - protein, 9 aa, synthetic construct
GGTGDDAAL

SEQ ID NO: 16187 - protein, 9 aa, synthetic construct
GGAGHDDMF

SEQ ID NO: 16188 - protein, 9 aa, synthetic construct
GGTGEDLLV

SEQ ID NO: 16189 - protein, 9 aa, synthetic construct
GGAGNDRAV

SEQ ID NO: 16190 - protein, 9 aa, synthetic construct
GGFGSDRIN

SEQ ID NO: 16191 - protein, 9 aa, synthetic construct
GGSGDDRVW

SEQ ID NO: 16192 - protein, 9 aa, synthetic construct
GGSGDDRVY

SEQ ID NO: 16193 - protein, 9 aa, synthetic construct
GGAGHDALF

SEQ ID NO: 16194 - protein, 9 aa, synthetic construct
GGIGNDSVV

SEQ ID NO: 16195 - protein, 9 aa, synthetic construct
GGIGNDTMS

SEQ ID NO: 16196 - protein, 9 aa, synthetic construct
GGTGEDTFD

SEQ ID NO: 16197 - protein, 9 aa, synthetic construct
GGNGADYLS

SEQ ID NO: 16198 - protein, 9 aa, synthetic construct
GGSGDDQVY

SEQ ID NO: 16199 - protein, 9 aa, synthetic construct
GGTGEDTLS

SEQ ID NO: 16200 - protein, 9 aa, synthetic construct
GGTGEDTLF

SEQ ID NO: 16201 - protein, 9 aa, synthetic construct
GGSGDDRFN

SEQ ID NO: 16202 - protein, 9 aa, synthetic construct
GGEGNDKLK

SEQ ID NO: 16203 - protein, 9 aa, synthetic construct
GGIGNDSVH

SEQ ID NO: 16204 - protein, 9 aa, synthetic construct
GGNGEDTLF

SEQ ID NO: 16205 - protein, 9 aa, synthetic construct
GGSGDDRIA

SEQ ID NO: 16206 - protein, 9 aa, synthetic construct
GGAGGDYVD

SEQ ID NO: 16207 - protein, 9 aa, synthetic construct
GGFGADSLV

SEQ ID NO: 16208 - protein, 9 aa, synthetic construct
GGSGDDRIF

SEQ ID NO: 16209 - protein, 9 aa, synthetic construct
GGAGHDTYV

SEQ ID NO: 16210 - protein, 9 aa, synthetic construct
GGAGNDRFM

SEQ ID NO: 16211 - protein, 9 aa, synthetic construct
GGSGDDRII

SEQ ID NO: 16212 - protein, 9 aa, synthetic construct
GGSGDDRIK

SEQ ID NO: 16213 - protein, 9 aa, synthetic construct
GGTGEDTIF

SEQ ID NO: 16214 - protein, 9 aa, synthetic construct
GGFGQDVLI

SEQ ID NO: 16215 - protein, 9 aa, synthetic construct
GGEGNDKLI

SEQ ID NO: 16216 - protein, 9 aa, synthetic construct
GGFGADTID

SEQ ID NO: 16217 - protein, 9 aa, synthetic construct
GGDGDDIVT

SEQ ID NO: 16218 - protein, 9 aa, synthetic construct
GGFGDDIYL

SEQ ID NO: 16219 - protein, 9 aa, synthetic construct
GGKGNDGLS

SEQ ID NO: 16220 - protein, 9 aa, synthetic construct
GGAGNDQVA

SEQ ID NO: 16221 - protein, 9 aa, synthetic construct
GGSGGDVLI

SEQ ID NO: 16222 - protein, 9 aa, synthetic construct
GGKGNDTVI

SEQ ID NO: 16223 - protein, 9 aa, synthetic construct
GGKGNDTVH

SEQ ID NO: 16224 - protein, 9 aa, synthetic construct
GGKGNDTMT

SEQ ID NO: 16225 - protein, 9 aa, synthetic construct
GGAGNDQMS

SEQ ID NO: 16226 - protein, 9 aa, synthetic construct
GGAGNDKFY

SEQ ID NO: 16227 - protein, 9 aa, synthetic construct
GGSGDDTAI

SEQ ID NO: 16228 - protein, 9 aa, synthetic construct
GGSGDDTAL

SEQ ID NO: 16229 - protein, 9 aa, synthetic construct
GGTGDDWLV

SEQ ID NO: 16230 - protein, 9 aa, synthetic construct
GGTGDDWLT

SEQ ID NO: 16231 - protein, 9 aa, synthetic construct
GGEGIDSMS

SEQ ID NO: 16232 - protein, 9 aa, synthetic construct
GGGGNDNIN

SEQ ID NO: 16233 - protein, 9 aa, synthetic construct
GGGGGDRLS

SEQ ID NO: 16234 - protein, 9 aa, synthetic construct
GGSGDDTFL

SEQ ID NO: 16235 - protein, 9 aa, synthetic construct
GGEGDDSYY

SEQ ID NO: 16236 - protein, 9 aa, synthetic construct
GGDGNDRAF

SEQ ID NO: 16237 - protein, 9 aa, synthetic construct
GGSGDDTFT

SEQ ID NO: 16238 - protein, 9 aa, synthetic construct
GGAGHDTLW

SEQ ID NO: 16239 - protein, 9 aa, synthetic construct
GGTGDDYME

SEQ ID NO: 16240 - protein, 9 aa, synthetic construct
GGNGDDFIF

SEQ ID NO: 16241 - protein, 9 aa, synthetic construct
GGFGADTLN

SEQ ID NO: 16242 - protein, 9 aa, synthetic construct
GGSGDDSII

SEQ ID NO: 16243 - protein, 9 aa, synthetic construct
GGKGNDVIA

SEQ ID NO: 16244 - protein, 9 aa, synthetic construct
GGEGIDRVS

SEQ ID NO: 16245 - protein, 9 aa, synthetic construct
GGAGHDTMT

SEQ ID NO: 16246 - protein, 9 aa, synthetic construct
GGDGNDNIN

SEQ ID NO: 16247 - protein, 9 aa, synthetic construct
GGAGHDEID

SEQ ID NO: 16248 - protein, 9 aa, synthetic construct
GGFGDDIVY

SEQ ID NO: 16249 - protein, 9 aa, synthetic construct
GGFGSDMLT

SEQ ID NO: 16250 - protein, 9 aa, synthetic construct
GGTGEDIVT

SEQ ID NO: 16251 - protein, 9 aa, synthetic construct
GGLGSDVFK

SEQ ID NO: 16252 - protein, 9 aa, synthetic construct
GGSGDDSMG

SEQ ID NO: 16253 - protein, 9 aa, synthetic construct
GGSGDDSIT

SEQ ID NO: 16254 - protein, 9 aa, synthetic construct
GGAGNDIYT

SEQ ID NO: 16255 - protein, 9 aa, synthetic construct
GGFGADTLA

SEQ ID NO: 16256 - protein, 9 aa, synthetic construct
GGAGHDFLF

SEQ ID NO: 16257 - protein, 9 aa, synthetic construct
GGFGADTLE

SEQ ID NO: 16258 - protein, 9 aa, synthetic construct
GGTGEDELK

SEQ ID NO: 16259 - protein, 9 aa, synthetic construct
GGAGHDFVW

SEQ ID NO: 16260 - protein, 9 aa, synthetic construct
GGTGDDALD

SEQ ID NO: 16261 - protein, 9 aa, synthetic construct
GGSGGDRLW

SEQ ID NO: 16262 - protein, 9 aa, synthetic construct
GGDGDDIYY

SEQ ID NO: 16263 - protein, 9 aa, synthetic construct
GGAGNDKLM

SEQ ID NO: 16264 - protein, 9 aa, synthetic construct
GGKGNDMLD

SEQ ID NO: 16265 - protein, 9 aa, synthetic construct
GGSGFDILD

SEQ ID NO: 16266 - protein, 9 aa, synthetic construct
GGTGDDLLM

SEQ ID NO: 16267 - protein, 9 aa, synthetic construct
GGTGDDLIV

SEQ ID NO: 16268 - protein, 9 aa, synthetic construct
GGAGNDLAY

SEQ ID NO: 16269 - protein, 9 aa, synthetic construct
GGSGFDKLF

SEQ ID NO: 16270 - protein, 9 aa, synthetic construct
GGSGFDLLD

SEQ ID NO: 16271 - protein, 9 aa, synthetic construct
GGAGNDLVT

SEQ ID NO: 16272 - protein, 9 aa, synthetic construct
GGTGDDLIR

SEQ ID NO: 16273 - protein, 9 aa, synthetic construct
GGSGFDLLS

SEQ ID NO: 16274 - protein, 9 aa, synthetic construct
GGFGDDELT

SEQ ID NO: 16275 - protein, 9 aa, synthetic construct
GGTGDDLIL

SEQ ID NO: 16276 - protein, 9 aa, synthetic construct
GGAGNDLVQ

SEQ ID NO: 16277 - protein, 9 aa, synthetic construct
GGDGRDELS

SEQ ID NO: 16278 - protein, 9 aa, synthetic construct
GGSGFDQFT

SEQ ID NO: 16279 - protein, 9 aa, synthetic construct
GGTGDDLIE

SEQ ID NO: 16280 - protein, 9 aa, synthetic construct
GGSGFDRFT

SEQ ID NO: 16281 - protein, 9 aa, synthetic construct
GGAGNDLVA

SEQ ID NO: 16282 - protein, 9 aa, synthetic construct
GGAGNDLFR

SEQ ID NO: 16283 - protein, 9 aa, synthetic construct
GGNGDDDLR

SEQ ID NO: 16284 - protein, 9 aa, synthetic construct
GGSGFDFLS

SEQ ID NO: 16285 - protein, 9 aa, synthetic construct
GGSGFDELW

SEQ ID NO: 16286 - protein, 9 aa, synthetic construct
GGEGIDTFS

SEQ ID NO: 16287 - protein, 9 aa, synthetic construct
GGKGNDMLF

SEQ ID NO: 16288 - protein, 9 aa, synthetic construct
GGAGNDMIR

SEQ ID NO: 16289 - protein, 9 aa, synthetic construct
GGFGRDLMR

SEQ ID NO: 16290 - protein, 9 aa, synthetic construct
GGSGEDVLI

SEQ ID NO: 16291 - protein, 9 aa, synthetic construct
GGAGHDQLS

SEQ ID NO: 16292 - protein, 9 aa, synthetic construct
GGSGEDVLL

SEQ ID NO: 16293 - protein, 9 aa, synthetic construct
GGDGNDQIY

SEQ ID NO: 16294 - protein, 9 aa, synthetic construct
GGAGHDQLT

SEQ ID NO: 16295 - protein, 9 aa, synthetic construct
GGTGDDLMY

SEQ ID NO: 16296 - protein, 9 aa, synthetic construct
GGTGDDLMT

SEQ ID NO: 16297 - protein, 9 aa, synthetic construct
GGSGEDWLD

SEQ ID NO: 16298 - protein, 9 aa, synthetic construct
GGGGGDKLL

SEQ ID NO: 16299 - protein, 9 aa, synthetic construct
GGEGNDIIV

SEQ ID NO: 16300 - protein, 9 aa, synthetic construct
GGSGGDKLF

SEQ ID NO: 16301 - protein, 9 aa, synthetic construct
GGEGIDTYT

SEQ ID NO: 16302 - protein, 9 aa, synthetic construct
GGTGDDLMF

SEQ ID NO: 16303 - protein, 9 aa, synthetic construct
GGEGIDWLW

SEQ ID NO: 16304 - protein, 9 aa, synthetic construct
GGKGNDMLL

SEQ ID NO: 16305 - protein, 9 aa, synthetic construct
GGTGDDFMD

SEQ ID NO: 16306 - protein, 9 aa, synthetic construct
GGKGNDKLD

SEQ ID NO: 16307 - protein, 9 aa, synthetic construct
GGAGHDRIS

SEQ ID NO: 16308 - protein, 9 aa, synthetic construct
GGSGFDSLY

SEQ ID NO: 16309 - protein, 9 aa, synthetic construct
GGDGRDILF

SEQ ID NO: 16310 - protein, 9 aa, synthetic construct
GGGGNDVFW

SEQ ID NO: 16311 - protein, 9 aa, synthetic construct
GGTGDDILY

SEQ ID NO: 16312 - protein, 9 aa, synthetic construct
GGFGDDFMS

SEQ ID NO: 16313 - protein, 9 aa, synthetic construct
GGDGDDKLR

SEQ ID NO: 16314 - protein, 9 aa, synthetic construct
GGDGRDFLY

SEQ ID NO: 16315 - protein, 9 aa, synthetic construct
GGLGSDIMT

SEQ ID NO: 16316 - protein, 9 aa, synthetic construct
GGKGNDLID

SEQ ID NO: 16317 - protein, 9 aa, synthetic construct
GGDGRDFLA

SEQ ID NO: 16318 - protein, 9 aa, synthetic construct
GGKGNDLLA

SEQ ID NO: 16319 - protein, 9 aa, synthetic construct
GGSGFDYYD

SEQ ID NO: 16320 - protein, 9 aa, synthetic construct
GGTGDDHIW

SEQ ID NO: 16321 - protein, 9 aa, synthetic construct
GGEGNDIIE

SEQ ID NO: 16322 - protein, 9 aa, synthetic construct
GGTGDDIIN

SEQ ID NO: 16323 - protein, 9 aa, synthetic construct
GGTGDDIFV

SEQ ID NO: 16324 - protein, 9 aa, synthetic construct
GGSGGDALF

SEQ ID NO: 16325 - protein, 9 aa, synthetic construct
GGLGSDIMI

SEQ ID NO: 16326 - protein, 9 aa, synthetic construct
GGTGDDHLE

SEQ ID NO: 16327 - protein, 9 aa, synthetic construct
GGTGDDHLR

SEQ ID NO: 16328 - protein, 9 aa, synthetic construct
GGAGHDSIS

SEQ ID NO: 16329 - protein, 9 aa, synthetic construct
GGDGRDFLN

SEQ ID NO: 16330 - protein, 9 aa, synthetic construct
GGSGFDVLN

SEQ ID NO: 16331 - protein, 9 aa, synthetic construct
GGGGNDVFS

SEQ ID NO: 16332 - protein, 9 aa, synthetic construct
GGTGDDIVF

SEQ ID NO: 16333 - protein, 9 aa, synthetic construct
GGEGADTML

SEQ ID NO: 16334 - protein, 9 aa, synthetic construct
GGAGHDRLH

SEQ ID NO: 16335 - protein, 9 aa, synthetic construct
GGSGGDHLY

SEQ ID NO: 16336 - protein, 9 aa, synthetic construct
GGNGDDEIH

SEQ ID NO: 16337 - protein, 9 aa, synthetic construct
GGSGFDTFV

SEQ ID NO: 16338 - protein, 9 aa, synthetic construct
GGAGNDLMM

SEQ ID NO: 16339 - protein, 9 aa, synthetic construct
GGAGNDLML

SEQ ID NO: 16340 - protein, 9 aa, synthetic construct
GGTGDDGFN

SEQ ID NO: 16341 - protein, 9 aa, synthetic construct
GGTGDDKLR

SEQ ID NO: 16342 - protein, 9 aa, synthetic construct
GGSGGDGLV

SEQ ID NO: 16343 - protein, 9 aa, synthetic construct
GGFGDDHLE

SEQ ID NO: 16344 - protein, 9 aa, synthetic construct
GGTGDDKLD

SEQ ID NO: 16345 - protein, 9 aa, synthetic construct
GGTGDDKLA

SEQ ID NO: 16346 - protein, 9 aa, synthetic construct
GGSGFDTLR

SEQ ID NO: 16347 - protein, 9 aa, synthetic construct
GGTGDDKIF

SEQ ID NO: 16348 - protein, 9 aa, synthetic construct
GGSGFDTLV

SEQ ID NO: 16349 - protein, 9 aa, synthetic construct
GGTGDDIYY

SEQ ID NO: 16350 - protein, 9 aa, synthetic construct
GGDGRDHVR

SEQ ID NO: 16351 - protein, 9 aa, synthetic construct
GGSGFDTYL

SEQ ID NO: 16352 - protein, 9 aa, synthetic construct
GGKGNDNYL

SEQ ID NO: 16353 - protein, 9 aa, synthetic construct
GGIGPDTIY

SEQ ID NO: 16354 - protein, 9 aa, synthetic construct
GGDGDDKLI

SEQ ID NO: 16355 - protein, 9 aa, synthetic construct
GGTGDDQLD

SEQ ID NO: 16356 - protein, 9 aa, synthetic construct
GGTGDDFIF

SEQ ID NO: 16357 - protein, 9 aa, synthetic construct
GGSGEDELI

SEQ ID NO: 16358 - protein, 9 aa, synthetic construct
GGTGDDRID

SEQ ID NO: 16359 - protein, 9 aa, synthetic construct
GGAGNDKMF

SEQ ID NO: 16360 - protein, 9 aa, synthetic construct
GGAGNDNLK

SEQ ID NO: 16361 - protein, 9 aa, synthetic construct
GGLGSDILD

SEQ ID NO: 16362 - protein, 9 aa, synthetic construct
GGKGNDRMS

SEQ ID NO: 16363 - protein, 9 aa, synthetic construct
GGNGDDELR

SEQ ID NO: 16364 - protein, 9 aa, synthetic construct
GGDGNDQVF

SEQ ID NO: 16365 - protein, 9 aa, synthetic construct
GGNGEDLVQ

SEQ ID NO: 16366 - protein, 9 aa, synthetic construct
GGEGADTMV

SEQ ID NO: 16367 - protein, 9 aa, synthetic construct
GGGGGDRLI

SEQ ID NO: 16368 - protein, 9 aa, synthetic construct
GGSGGDQID

SEQ ID NO: 16369 - protein, 9 aa, synthetic construct
GGTGDDQLW

SEQ ID NO: 16370 - protein, 9 aa, synthetic construct
GGTGDDFLD

SEQ ID NO: 16371 - protein, 9 aa, synthetic construct
GGTGDDFLF

SEQ ID NO: 16372 - protein, 9 aa, synthetic construct
GGDGDDKIS

SEQ ID NO: 16373 - protein, 9 aa, synthetic construct
GGNGDDDFV

SEQ ID NO: 16374 - protein, 9 aa, synthetic construct
GGTGDDQLL

SEQ ID NO: 16375 - protein, 9 aa, synthetic construct
GGKGNDRYL

SEQ ID NO: 16376 - protein, 9 aa, synthetic construct
GGDGNDNVN

SEQ ID NO: 16377 - protein, 9 aa, synthetic construct
GGDGDDQVW

SEQ ID NO: 16378 - protein, 9 aa, synthetic construct
GGSGDDYME

SEQ ID NO: 16379 - protein, 9 aa, synthetic construct
GGSGDDYIS

SEQ ID NO: 16380 - protein, 9 aa, synthetic construct
GGTGDDRLQ

SEQ ID NO: 16381 - protein, 9 aa, synthetic construct
GGKGNDSLV

SEQ ID NO: 16382 - protein, 9 aa, synthetic construct
GGSGDDYLI

SEQ ID NO: 16383 - protein, 9 aa, synthetic construct
GGAGHDTIL

SEQ ID NO: 16384 - protein, 9 aa, synthetic construct
GGSGDDYLR

SEQ ID NO: 16385 - protein, 9 aa, synthetic construct
GGAGHDLLQ

SEQ ID NO: 16386 - protein, 9 aa, synthetic construct
GGSGDDYLY

SEQ ID NO: 16387 - protein, 9 aa, synthetic construct
GGTGDDEMY

SEQ ID NO: 16388 - protein, 9 aa, synthetic construct
GGAGHDLLV

SEQ ID NO: 16389 - protein, 9 aa, synthetic construct
GGGGGDRLL

SEQ ID NO: 16390 - protein, 9 aa, synthetic construct
GGAGHDLLT

SEQ ID NO: 16391 - protein, 9 aa, synthetic construct
GGAGNDNML

SEQ ID NO: 16392 - protein, 9 aa, synthetic construct
GGSGDDYVH

SEQ ID NO: 16393 - protein, 9 aa, synthetic construct
GGAGHDTIE

SEQ ID NO: 16394 - protein, 9 aa, synthetic construct
GGAGNDNMD

SEQ ID NO: 16395 - protein, 9 aa, synthetic construct
GGTGDDFID

SEQ ID NO: 16396 - protein, 9 aa, synthetic construct
GGSGGDRIF

SEQ ID NO: 16397 - protein, 9 aa, synthetic construct
GGEGNDILM

SEQ ID NO: 16398 - protein, 9 aa, synthetic construct
GGNGDDELH

SEQ ID NO: 16399 - protein, 9 aa, synthetic construct
GGTGDDLVF

SEQ ID NO: 16400 - protein, 9 aa, synthetic construct
GGEGIDTLD

SEQ ID NO: 16401 - protein, 9 aa, synthetic construct
GGGGNDNLT

SEQ ID NO: 16402 - protein, 9 aa, synthetic construct
GGIGNDYLN

SEQ ID NO: 16403 - protein, 9 aa, synthetic construct
GGAGNDKVL

SEQ ID NO: 16404 - protein, 9 aa, synthetic construct
GGAGNDKVY

SEQ ID NO: 16405 - protein, 9 aa, synthetic construct
GGSGEDSLV

SEQ ID NO: 16406 - protein, 9 aa, synthetic construct
GGTGDDMLA

SEQ ID NO: 16407 - protein, 9 aa, synthetic construct
GGNGDDDIT

SEQ ID NO: 16408 - protein, 9 aa, synthetic construct
GGSGGDLLF

SEQ ID NO: 16409 - protein, 9 aa, synthetic construct
GGFGDDEID

SEQ ID NO: 16410 - protein, 9 aa, synthetic construct
GGAGHDQLD

SEQ ID NO: 16411 - protein, 9 aa, synthetic construct
GGTGDDLYV

SEQ ID NO: 16412 - protein, 9 aa, synthetic construct
GGAGHDQLE

SEQ ID NO: 16413 - protein, 9 aa, synthetic construct
GGDGNDQIR

SEQ ID NO: 16414 - protein, 9 aa, synthetic construct
GGLGSDTME

SEQ ID NO: 16415 - protein, 9 aa, synthetic construct
GGIGRDGAK

SEQ ID NO: 16416 - protein, 9 aa, synthetic construct
GGNGDDDLF

SEQ ID NO: 16417 - protein, 9 aa, synthetic construct
GGFGDDELH

SEQ ID NO: 16418 - protein, 9 aa, synthetic construct
GGAGHDQLM

SEQ ID NO: 16419 - protein, 9 aa, synthetic construct
GGTGDDLVI

SEQ ID NO: 16420 - protein, 9 aa, synthetic construct
GGKGNDKFV

SEQ ID NO: 16421 - protein, 9 aa, synthetic construct
GGGGNDVIG

SEQ ID NO: 16422 - protein, 9 aa, synthetic construct
GGEGIDTLS

SEQ ID NO: 16423 - protein, 9 aa, synthetic construct
GGIGNDWLY

SEQ ID NO: 16424 - protein, 9 aa, synthetic construct
GGDGNDQAY

SEQ ID NO: 16425 - protein, 9 aa, synthetic construct
GGTGDDQID

SEQ ID NO: 16426 - protein, 9 aa, synthetic construct
GGNGEDLIY

SEQ ID NO: 16427 - protein, 9 aa, synthetic construct
GGLGSDTMR

SEQ ID NO: 16428 - protein, 9 aa, synthetic construct
GGGGNDNLR

SEQ ID NO: 16429 - protein, 9 aa, synthetic construct
GGLGSDILL

SEQ ID NO: 16430 - protein, 9 aa, synthetic construct
GGSGEDMLF

SEQ ID NO: 16431 - protein, 9 aa, synthetic construct
GGAGHDMLI

SEQ ID NO: 16432 - protein, 9 aa, synthetic construct
GGNGDDELF

SEQ ID NO: 16433 - protein, 9 aa, synthetic construct
GGKGNDIYY

SEQ ID NO: 16434 - protein, 9 aa, synthetic construct
GGSGEDNLH

SEQ ID NO: 16435 - protein, 9 aa, synthetic construct
GGEGIDTLL

SEQ ID NO: 16436 - protein, 9 aa, synthetic construct
GGTGDDFLR

SEQ ID NO: 16437 - protein, 9 aa, synthetic construct
GGAGNDMMS

SEQ ID NO: 16438 - protein, 9 aa, synthetic construct
GGTGDDFLS

SEQ ID NO: 16439 - protein, 9 aa, synthetic construct
GGAGNDKVD

SEQ ID NO: 16440 - protein, 9 aa, synthetic construct
GGTGDDNLI

SEQ ID NO: 16441 - protein, 9 aa, synthetic construct
GGSGEDRLY

SEQ ID NO: 16442 - protein, 9 aa, synthetic construct
GGSGDDQVF

SEQ ID NO: 16443 - protein, 9 aa, synthetic construct
GGSGDDQLV

SEQ ID NO: 16444 - protein, 9 aa, synthetic construct
GGTGKDKLT

SEQ ID NO: 16445 - protein, 9 aa, synthetic construct
GGKGRDILT

SEQ ID NO: 16446 - protein, 9 aa, synthetic construct
GGAGNDTAI

SEQ ID NO: 16447 - protein, 9 aa, synthetic construct
GGTGHDTMA

SEQ ID NO: 16448 - protein, 9 aa, synthetic construct
GGSGHDSLF

SEQ ID NO: 16449 - protein, 9 aa, synthetic construct
GGNGFDHLD

SEQ ID NO: 16450 - protein, 9 aa, synthetic construct
GGAGNDTAF

SEQ ID NO: 16451 - protein, 9 aa, synthetic construct
GGSGADYMV

SEQ ID NO: 16452 - protein, 9 aa, synthetic construct
GGDGNDLVH

SEQ ID NO: 16453 - protein, 9 aa, synthetic construct
GGTGHDTLL

SEQ ID NO: 16454 - protein, 9 aa, synthetic construct
GGSGDDAAS

SEQ ID NO: 16455 - protein, 9 aa, synthetic construct
GGEGIDLLR

SEQ ID NO: 16456 - protein, 9 aa, synthetic construct
GGSGDDAIA

SEQ ID NO: 16457 - protein, 9 aa, synthetic construct
GGTGHDTLF

SEQ ID NO: 16458 - protein, 9 aa, synthetic construct
GGSGDDAIN

SEQ ID NO: 16459 - protein, 9 aa, synthetic construct
GGSGHDSLD

SEQ ID NO: 16460 - protein, 9 aa, synthetic construct
GGTGHDTLE

SEQ ID NO: 16461 - protein, 9 aa, synthetic construct
GGDGDDIMD

SEQ ID NO: 16462 - protein, 9 aa, synthetic construct
GGTGHDTIT

SEQ ID NO: 16463 - protein, 9 aa, synthetic construct
GGEGADYIG

SEQ ID NO: 16464 - protein, 9 aa, synthetic construct
GGSGDDALE

SEQ ID NO: 16465 - protein, 9 aa, synthetic construct
GGEGDDMLN

SEQ ID NO: 16466 - protein, 9 aa, synthetic construct
GGSGADYLD

SEQ ID NO: 16467 - protein, 9 aa, synthetic construct
GGAGGDLLT

SEQ ID NO: 16468 - protein, 9 aa, synthetic construct
GGKGNDEIS

SEQ ID NO: 16469 - protein, 9 aa, synthetic construct
GGDGNDLMS

SEQ ID NO: 16470 - protein, 9 aa, synthetic construct
GGIGNDILE

SEQ ID NO: 16471 - protein, 9 aa, synthetic construct
GGAGNDIFL

SEQ ID NO: 16472 - protein, 9 aa, synthetic construct
GGSGADVVA

SEQ ID NO: 16473 - protein, 9 aa, synthetic construct
GGSGHDSLY

SEQ ID NO: 16474 - protein, 9 aa, synthetic construct
GGAGGDMFV

SEQ ID NO: 16475 - protein, 9 aa, synthetic construct
GGAGGDMLF

SEQ ID NO: 16476 - protein, 9 aa, synthetic construct
GGTGHDVLV

SEQ ID NO: 16477 - protein, 9 aa, synthetic construct
GGSGADVYH

SEQ ID NO: 16478 - protein, 9 aa, synthetic construct
GGAGNDIFN

SEQ ID NO: 16479 - protein, 9 aa, synthetic construct
GGDGNDLVF

SEQ ID NO: 16480 - protein, 9 aa, synthetic construct
GGTGHDVLL

SEQ ID NO: 16481 - protein, 9 aa, synthetic construct
GGTGHDVLG

SEQ ID NO: 16482 - protein, 9 aa, synthetic construct
GGAGGDNID

SEQ ID NO: 16483 - protein, 9 aa, synthetic construct
GGAGNDIFQ

SEQ ID NO: 16484 - protein, 9 aa, synthetic construct
GGDGDDLAN

SEQ ID NO: 16485 - protein, 9 aa, synthetic construct
GGSGADYIE

SEQ ID NO: 16486 - protein, 9 aa, synthetic construct
GGLGSDEFV

SEQ ID NO: 16487 - protein, 9 aa, synthetic construct
GGAGNDTAY

SEQ ID NO: 16488 - protein, 9 aa, synthetic construct
GGSGDDALI

SEQ ID NO: 16489 - protein, 9 aa, synthetic construct
GGEGNDLLG

SEQ ID NO: 16490 - protein, 9 aa, synthetic construct
GGEGDDSYV

SEQ ID NO: 16491 - protein, 9 aa, synthetic construct
GGFGADAMD

SEQ ID NO: 16492 - protein, 9 aa, synthetic construct
GGDGQDTVS

SEQ ID NO: 16493 - protein, 9 aa, synthetic construct
GGFGADEIL

SEQ ID NO: 16494 - protein, 9 aa, synthetic construct
GGGGNDWLR

SEQ ID NO: 16495 - protein, 9 aa, synthetic construct
GGDGGDIYV

SEQ ID NO: 16496 - protein, 9 aa, synthetic construct
GGDGNDMAV

SEQ ID NO: 16497 - protein, 9 aa, synthetic construct
GGDGNDMFL

SEQ ID NO: 16498 - protein, 9 aa, synthetic construct
GGSGHDRLS

SEQ ID NO: 16499 - protein, 9 aa, synthetic construct
GGIGNDKLS

SEQ ID NO: 16500 - protein, 9 aa, synthetic construct
GGTGADTVL

SEQ ID NO: 16501 - protein, 9 aa, synthetic construct
GGFGSDTLV

SEQ ID NO: 16502 - protein, 9 aa, synthetic construct
GGSGHDRLL

SEQ ID NO: 16503 - protein, 9 aa, synthetic construct
GGAGGDRIN

SEQ ID NO: 16504 - protein, 9 aa, synthetic construct
GGSGDDEIT

SEQ ID NO: 16505 - protein, 9 aa, synthetic construct
GGTGHDLIY

SEQ ID NO: 16506 - protein, 9 aa, synthetic construct
GGAGGDRIR

SEQ ID NO: 16507 - protein, 9 aa, synthetic construct
GGDGRDSLE

SEQ ID NO: 16508 - protein, 9 aa, synthetic construct
GGNGDDFLS

SEQ ID NO: 16509 - protein, 9 aa, synthetic construct
GGTGHDILE

SEQ ID NO: 16510 - protein, 9 aa, synthetic construct
GGNGDDFLR

SEQ ID NO: 16511 - protein, 9 aa, synthetic construct
GGTGHDRIY

SEQ ID NO: 16512 - protein, 9 aa, synthetic construct
GGGGNDTMD

SEQ ID NO: 16513 - protein, 9 aa, synthetic construct
GGTGHDRLE

SEQ ID NO: 16514 - protein, 9 aa, synthetic construct
GGAGNDSVG

SEQ ID NO: 16515 - protein, 9 aa, synthetic construct
GGSGDDALV

SEQ ID NO: 16516 - protein, 9 aa, synthetic construct
GGAGGDQIL

SEQ ID NO: 16517 - protein, 9 aa, synthetic construct
GGAGNDSYF

SEQ ID NO: 16518 - protein, 9 aa, synthetic construct
GGTGHDSLV

SEQ ID NO: 16519 - protein, 9 aa, synthetic construct
GGAGGDQIS

SEQ ID NO: 16520 - protein, 9 aa, synthetic construct
GGAGGDQIY

SEQ ID NO: 16521 - protein, 9 aa, synthetic construct
GGSGDDAVS

SEQ ID NO: 16522 - protein, 9 aa, synthetic construct
GGTGHDSID

SEQ ID NO: 16523 - protein, 9 aa, synthetic construct
GGAGGDQLI

SEQ ID NO: 16524 - protein, 9 aa, synthetic construct
GGSGDDDLQ

SEQ ID NO: 16525 - protein, 9 aa, synthetic construct
GGFGSDTYL

SEQ ID NO: 16526 - protein, 9 aa, synthetic construct
GGTGHDRLY

SEQ ID NO: 16527 - protein, 9 aa, synthetic construct
GGAGGDQLN

SEQ ID NO: 16528 - protein, 9 aa, synthetic construct
GGLGSDFID

SEQ ID NO: 16529 - protein, 9 aa, synthetic construct
GGTGHDRLN

SEQ ID NO: 16530 - protein, 9 aa, synthetic construct
GGSGDDDLA

SEQ ID NO: 16531 - protein, 9 aa, synthetic construct
GGTGHDRLI

SEQ ID NO: 16532 - protein, 9 aa, synthetic construct
GGSGDDDLM

SEQ ID NO: 16533 - protein, 9 aa, synthetic construct
GGTGADTIW

SEQ ID NO: 16534 - protein, 9 aa, synthetic construct
GGIGNDILA

SEQ ID NO: 16535 - protein, 9 aa, synthetic construct
GGGGNDTVR

SEQ ID NO: 16536 - protein, 9 aa, synthetic construct
GGAGGDHFV

SEQ ID NO: 16537 - protein, 9 aa, synthetic construct
GGDGDDRVL

SEQ ID NO: 16538 - protein, 9 aa, synthetic construct
GGTGKDALV

SEQ ID NO: 16539 - protein, 9 aa, synthetic construct
GGSGADTFQ

SEQ ID NO: 16540 - protein, 9 aa, synthetic construct
GGTGKDALS

SEQ ID NO: 16541 - protein, 9 aa, synthetic construct
GGEGYDRLR

SEQ ID NO: 16542 - protein, 9 aa, synthetic construct
GGTGIDWLD

SEQ ID NO: 16543 - protein, 9 aa, synthetic construct
GGTGIDWAT

SEQ ID NO: 16544 - protein, 9 aa, synthetic construct
GGSGADTIA

SEQ ID NO: 16545 - protein, 9 aa, synthetic construct
GGTGIDVLS

SEQ ID NO: 16546 - protein, 9 aa, synthetic construct
GGFGSDVLV

SEQ ID NO: 16547 - protein, 9 aa, synthetic construct
GGFGQDSIS

SEQ ID NO: 16548 - protein, 9 aa, synthetic construct
GGIGNDELH

SEQ ID NO: 16549 - protein, 9 aa, synthetic construct
GGAGGDILA

SEQ ID NO: 16550 - protein, 9 aa, synthetic construct
GGSGHDTVY

SEQ ID NO: 16551 - protein, 9 aa, synthetic construct
GGIGNDELN

SEQ ID NO: 16552 - protein, 9 aa, synthetic construct
GGSGADTIV

SEQ ID NO: 16553 - protein, 9 aa, synthetic construct
GGLGSDTII

SEQ ID NO: 16554 - protein, 9 aa, synthetic construct
GGIGSDLLF

SEQ ID NO: 16555 - protein, 9 aa, synthetic construct
GGTGIDTLE

SEQ ID NO: 16556 - protein, 9 aa, synthetic construct
GGAGGDHLA

SEQ ID NO: 16557 - protein, 9 aa, synthetic construct
GGAGGDGLY

SEQ ID NO: 16558 - protein, 9 aa, synthetic construct
GGSGHDTFV

SEQ ID NO: 16559 - protein, 9 aa, synthetic construct
GGSGADTFG

SEQ ID NO: 16560 - protein, 9 aa, synthetic construct
GGNGADTLK

SEQ ID NO: 16561 - protein, 9 aa, synthetic construct
GGAGGDFLA

SEQ ID NO: 16562 - protein, 9 aa, synthetic construct
GGAGNDHMI

SEQ ID NO: 16563 - protein, 9 aa, synthetic construct
GGNGDDWLD

SEQ ID NO: 16564 - protein, 9 aa, synthetic construct
GGAGGDFLK

SEQ ID NO: 16565 - protein, 9 aa, synthetic construct
GGTGADSLW

SEQ ID NO: 16566 - protein, 9 aa, synthetic construct
GGTGKDILV

SEQ ID NO: 16567 - protein, 9 aa, synthetic construct
GGTGKDILT

SEQ ID NO: 16568 - protein, 9 aa, synthetic construct
GGAGGDFLS

SEQ ID NO: 16569 - protein, 9 aa, synthetic construct
GGGGNDYIY

SEQ ID NO: 16570 - protein, 9 aa, synthetic construct
GGGGNDYIV

SEQ ID NO: 16571 - protein, 9 aa, synthetic construct
GGSGADTAI

SEQ ID NO: 16572 - protein, 9 aa, synthetic construct
GGTGKDILA

SEQ ID NO: 16573 - protein, 9 aa, synthetic construct
GGFGQDLIH

SEQ ID NO: 16574 - protein, 9 aa, synthetic construct
GGAGNDHVI

SEQ ID NO: 16575 - protein, 9 aa, synthetic construct
GGTGKDIFV

SEQ ID NO: 16576 - protein, 9 aa, synthetic construct
GGEGYDNIF

SEQ ID NO: 16577 - protein, 9 aa, synthetic construct
GGTGADSMK

SEQ ID NO: 16578 - protein, 9 aa, synthetic construct
GGTGADSML

SEQ ID NO: 16579 - protein, 9 aa, synthetic construct
GGSGADTLM

SEQ ID NO: 16580 - protein, 9 aa, synthetic construct
GGTGIDTIY

SEQ ID NO: 16581 - protein, 9 aa, synthetic construct
GGDGRDTIY

SEQ ID NO: 16582 - protein, 9 aa, synthetic construct
GGGGHDTLV

SEQ ID NO: 16583 - protein, 9 aa, synthetic construct
GGDGDDLAS

SEQ ID NO: 16584 - protein, 9 aa, synthetic construct
GGLGSDTIR

SEQ ID NO: 16585 - protein, 9 aa, synthetic construct
GGSGADVFL

SEQ ID NO: 16586 - protein, 9 aa, synthetic construct
GGAGGDLID

SEQ ID NO: 16587 - protein, 9 aa, synthetic construct
GGAGGDLIE

SEQ ID NO: 16588 - protein, 9 aa, synthetic construct
GGDGNDLMF

SEQ ID NO: 16589 - protein, 9 aa, synthetic construct
GGSGHDTIY

SEQ ID NO: 16590 - protein, 9 aa, synthetic construct
GGTGIDLLF

SEQ ID NO: 16591 - protein, 9 aa, synthetic construct
GGKGRDNLN

SEQ ID NO: 16592 - protein, 9 aa, synthetic construct
GGAGNDIAY

SEQ ID NO: 16593 - protein, 9 aa, synthetic construct
GGIGSDILV

SEQ ID NO: 16594 - protein, 9 aa, synthetic construct
GGTGIDLLD

SEQ ID NO: 16595 - protein, 9 aa, synthetic construct
GGIGNDIIE

SEQ ID NO: 16596 - protein, 9 aa, synthetic construct
GGTGIDKIS

SEQ ID NO: 16597 - protein, 9 aa, synthetic construct
GGDGRDTFL

SEQ ID NO: 16598 - protein, 9 aa, synthetic construct
GGAGNDIFA

SEQ ID NO: 16599 - protein, 9 aa, synthetic construct
GGEGNDHMS

SEQ ID NO: 16600 - protein, 9 aa, synthetic construct
GGTGIDIFR

SEQ ID NO: 16601 - protein, 9 aa, synthetic construct
GGTGIDHMQ

SEQ ID NO: 16602 - protein, 9 aa, synthetic construct
GGIGNDIFQ

SEQ ID NO: 16603 - protein, 9 aa, synthetic construct
GGSGHDTLH

SEQ ID NO: 16604 - protein, 9 aa, synthetic construct
GGIGNDHYE

SEQ ID NO: 16605 - protein, 9 aa, synthetic construct
GGNGADTVD

SEQ ID NO: 16606 - protein, 9 aa, synthetic construct
GGIGNDFLA

SEQ ID NO: 16607 - protein, 9 aa, synthetic construct
GGSGHDTMT

SEQ ID NO: 16608 - protein, 9 aa, synthetic construct
GGEGKDIIG

SEQ ID NO: 16609 - protein, 9 aa, synthetic construct
GGSGADTME

SEQ ID NO: 16610 - protein, 9 aa, synthetic construct
GGTGADTAL

SEQ ID NO: 16611 - protein, 9 aa, synthetic construct
GGIGNDFLY

SEQ ID NO: 16612 - protein, 9 aa, synthetic construct
GGTGIDSLV

SEQ ID NO: 16613 - protein, 9 aa, synthetic construct
GGNGADTMR

SEQ ID NO: 16614 - protein, 9 aa, synthetic construct
GGIGNDGLF

SEQ ID NO: 16615 - protein, 9 aa, synthetic construct
GGIGNDHLY

SEQ ID NO: 16616 - protein, 9 aa, synthetic construct
GGIGNDGLS

SEQ ID NO: 16617 - protein, 9 aa, synthetic construct
GGSGADTVS

SEQ ID NO: 16618 - protein, 9 aa, synthetic construct
GGDGFDTAV

SEQ ID NO: 16619 - protein, 9 aa, synthetic construct
GGSGADTVY

SEQ ID NO: 16620 - protein, 9 aa, synthetic construct
GGSGHDTLL

SEQ ID NO: 16621 - protein, 9 aa, synthetic construct
GGSGHDTLK

SEQ ID NO: 16622 - protein, 9 aa, synthetic construct
GGDGRDTIF

SEQ ID NO: 16623 - protein, 9 aa, synthetic construct
GGDGDDRMT

SEQ ID NO: 16624 - protein, 9 aa, synthetic construct
GGTGHDHLF

SEQ ID NO: 16625 - protein, 9 aa, synthetic construct
GGAGGDRLT

SEQ ID NO: 16626 - protein, 9 aa, synthetic construct
GGTGHDELQ

SEQ ID NO: 16627 - protein, 9 aa, synthetic construct
GGDGNDNFI

SEQ ID NO: 16628 - protein, 9 aa, synthetic construct
GGIGNDRLN

SEQ ID NO: 16629 - protein, 9 aa, synthetic construct
GGAGGDVID

SEQ ID NO: 16630 - protein, 9 aa, synthetic construct
GGIGNDRLS

SEQ ID NO: 16631 - protein, 9 aa, synthetic construct
GGIGNDRLT

SEQ ID NO: 16632 - protein, 9 aa, synthetic construct
GGKGNDWID

SEQ ID NO: 16633 - protein, 9 aa, synthetic construct
GGIGNDRLW

SEQ ID NO: 16634 - protein, 9 aa, synthetic construct
GGSGDDLMS

SEQ ID NO: 16635 - protein, 9 aa, synthetic construct
GGTGFDVFE

SEQ ID NO: 16636 - protein, 9 aa, synthetic construct
GGTGFDVAQ

SEQ ID NO: 16637 - protein, 9 aa, synthetic construct
GGKGNDVYR

SEQ ID NO: 16638 - protein, 9 aa, synthetic construct
GGAGGDVLF

SEQ ID NO: 16639 - protein, 9 aa, synthetic construct
GGSGDDLVQ

SEQ ID NO: 16640 - protein, 9 aa, synthetic construct
GGSGDDLVV

SEQ ID NO: 16641 - protein, 9 aa, synthetic construct
GGKGNDVMT

SEQ ID NO: 16642 - protein, 9 aa, synthetic construct
GGSGDDLYI

SEQ ID NO: 16643 - protein, 9 aa, synthetic construct
GGGGNDVVR

SEQ ID NO: 16644 - protein, 9 aa, synthetic construct
GGEGNDKLS

SEQ ID NO: 16645 - protein, 9 aa, synthetic construct
GGSGDDLYV

SEQ ID NO: 16646 - protein, 9 aa, synthetic construct
GGGGNDMLY

SEQ ID NO: 16647 - protein, 9 aa, synthetic construct
GGTGGDDIN

SEQ ID NO: 16648 - protein, 9 aa, synthetic construct
GGIGNDRLL

SEQ ID NO: 16649 - protein, 9 aa, synthetic construct
GGEGNDLIQ

SEQ ID NO: 16650 - protein, 9 aa, synthetic construct
GGAGGDVFK

SEQ ID NO: 16651 - protein, 9 aa, synthetic construct
GGNGEDTLN

SEQ ID NO: 16652 - protein, 9 aa, synthetic construct
GGSGDDLAY

SEQ ID NO: 16653 - protein, 9 aa, synthetic construct
GGAGNDRVH

SEQ ID NO: 16654 - protein, 9 aa, synthetic construct
GGAGGDTMY

SEQ ID NO: 16655 - protein, 9 aa, synthetic construct
GGAGGDTVD

SEQ ID NO: 16656 - protein, 9 aa, synthetic construct
GGTGGDILN

SEQ ID NO: 16657 - protein, 9 aa, synthetic construct
GGLGSDVLF

SEQ ID NO: 16658 - protein, 9 aa, synthetic construct
GGFGADLLN

SEQ ID NO: 16659 - protein, 9 aa, synthetic construct
GGKGNDWLR

SEQ ID NO: 16660 - protein, 9 aa, synthetic construct
GGTGADWLV

SEQ ID NO: 16661 - protein, 9 aa, synthetic construct
GGAGNDIMI

SEQ ID NO: 16662 - protein, 9 aa, synthetic construct
GGTGGDIFV

SEQ ID NO: 16663 - protein, 9 aa, synthetic construct
GGTGADWME

SEQ ID NO: 16664 - protein, 9 aa, synthetic construct
GGGGGDRLW

SEQ ID NO: 16665 - protein, 9 aa, synthetic construct
GGFGADLLS

SEQ ID NO: 16666 - protein, 9 aa, synthetic construct
GGDGRDRFA

SEQ ID NO: 16667 - protein, 9 aa, synthetic construct
GGIGNDRLA

SEQ ID NO: 16668 - protein, 9 aa, synthetic construct
GGDGNDRFT

SEQ ID NO: 16669 - protein, 9 aa, synthetic construct
GGIGNDRLH

SEQ ID NO: 16670 - protein, 9 aa, synthetic construct
GGAGNDRMF

SEQ ID NO: 16671 - protein, 9 aa, synthetic construct
GGTGFDTLD

SEQ ID NO: 16672 - protein, 9 aa, synthetic construct
GGSGHDFLT

SEQ ID NO: 16673 - protein, 9 aa, synthetic construct
GGLGSDVLE

SEQ ID NO: 16674 - protein, 9 aa, synthetic construct
GGDGDDKVF

SEQ ID NO: 16675 - protein, 9 aa, synthetic construct
GGTGEDWLA

SEQ ID NO: 16676 - protein, 9 aa, synthetic construct
GGFGADSLD

SEQ ID NO: 16677 - protein, 9 aa, synthetic construct
GGGGNDTVI

SEQ ID NO: 16678 - protein, 9 aa, synthetic construct
GGSGDDQII

SEQ ID NO: 16679 - protein, 9 aa, synthetic construct
GGSGDDQIQ

SEQ ID NO: 16680 - protein, 9 aa, synthetic construct
GGSGHDCLL

SEQ ID NO: 16681 - protein, 9 aa, synthetic construct
GGAGNDRIM

SEQ ID NO: 16682 - protein, 9 aa, synthetic construct
GGTGADYME

SEQ ID NO: 16683 - protein, 9 aa, synthetic construct
GGEGADVVT

SEQ ID NO: 16684 - protein, 9 aa, synthetic construct
GGTGEDVLI

SEQ ID NO: 16685 - protein, 9 aa, synthetic construct
GGGGNDVLW

SEQ ID NO: 16686 - protein, 9 aa, synthetic construct
GGAGGDYLI

SEQ ID NO: 16687 - protein, 9 aa, synthetic construct
GGSGDDQLI

SEQ ID NO: 16688 - protein, 9 aa, synthetic construct
GGSGDDQLK

SEQ ID NO: 16689 - protein, 9 aa, synthetic construct
GGIGNDSMD

SEQ ID NO: 16690 - protein, 9 aa, synthetic construct
GGSGDDQLN

SEQ ID NO: 16691 - protein, 9 aa, synthetic construct
GGAGGDYLL

SEQ ID NO: 16692 - protein, 9 aa, synthetic construct
GGIGNDSMH

SEQ ID NO: 16693 - protein, 9 aa, synthetic construct
GGFGADSIM

SEQ ID NO: 16694 - protein, 9 aa, synthetic construct
GGTGFDEAS

SEQ ID NO: 16695 - protein, 9 aa, synthetic construct
GGAGHDVFQ

SEQ ID NO: 16696 - protein, 9 aa, synthetic construct
GGKGNDVMI

SEQ ID NO: 16697 - protein, 9 aa, synthetic construct
GGFGADQLS

SEQ ID NO: 16698 - protein, 9 aa, synthetic construct
GGTGFDSLD

SEQ ID NO: 16699 - protein, 9 aa, synthetic construct
GGSGDDMLR

SEQ ID NO: 16700 - protein, 9 aa, synthetic construct
GGFGADQMA

SEQ ID NO: 16701 - protein, 9 aa, synthetic construct
GGSGDDMLT

SEQ ID NO: 16702 - protein, 9 aa, synthetic construct
GGIGNDRYV

SEQ ID NO: 16703 - protein, 9 aa, synthetic construct
GGLGSDTLE

SEQ ID NO: 16704 - protein, 9 aa, synthetic construct
GGTGFDRLT

SEQ ID NO: 16705 - protein, 9 aa, synthetic construct
GGSGDDNIT

SEQ ID NO: 16706 - protein, 9 aa, synthetic construct
GGIGNDSIT

SEQ ID NO: 16707 - protein, 9 aa, synthetic construct
GGFGADRFV

SEQ ID NO: 16708 - protein, 9 aa, synthetic construct
GGSGDDNLF

SEQ ID NO: 16709 - protein, 9 aa, synthetic construct
GGGGNDVMH

SEQ ID NO: 16710 - protein, 9 aa, synthetic construct
GGEGKDELT

SEQ ID NO: 16711 - protein, 9 aa, synthetic construct
GGSGDDNLS

SEQ ID NO: 16712 - protein, 9 aa, synthetic construct
GGAGNDIVK

SEQ ID NO: 16713 - protein, 9 aa, synthetic construct
GGGGGDRLV

SEQ ID NO: 16714 - protein, 9 aa, synthetic construct
GGSGHDDLS

SEQ ID NO: 16715 - protein, 9 aa, synthetic construct
GGAGHDVIF

SEQ ID NO: 16716 - protein, 9 aa, synthetic construct
GGAGGDTMT

SEQ ID NO: 16717 - protein, 9 aa, synthetic construct
GGFGSDSLY

SEQ ID NO: 16718 - protein, 9 aa, synthetic construct
GGIGNDMLD

SEQ ID NO: 16719 - protein, 9 aa, synthetic construct
GGEGNDLFV

SEQ ID NO: 16720 - protein, 9 aa, synthetic construct
GGFGSDTLT

SEQ ID NO: 16721 - protein, 9 aa, synthetic construct
GGTGGDTYV

SEQ ID NO: 16722 - protein, 9 aa, synthetic construct
GGNGEDVIR

SEQ ID NO: 16723 - protein, 9 aa, synthetic construct
GGTGADVIS

SEQ ID NO: 16724 - protein, 9 aa, synthetic construct
GGAGGDSVI

SEQ ID NO: 16725 - protein, 9 aa, synthetic construct
GGDGRDRLY

SEQ ID NO: 16726 - protein, 9 aa, synthetic construct
GGKGQDKLN

SEQ ID NO: 16727 - protein, 9 aa, synthetic construct
GGSGDDHIH

SEQ ID NO: 16728 - protein, 9 aa, synthetic construct
GGKGQDKLA

SEQ ID NO: 16729 - protein, 9 aa, synthetic construct
GGTGGDTLQ

SEQ ID NO: 16730 - protein, 9 aa, synthetic construct
GGTGADVIT

SEQ ID NO: 16731 - protein, 9 aa, synthetic construct
GGKGQDIFS

SEQ ID NO: 16732 - protein, 9 aa, synthetic construct
GGFGDDKVF

SEQ ID NO: 16733 - protein, 9 aa, synthetic construct
GGSGDDHLE

SEQ ID NO: 16734 - protein, 9 aa, synthetic construct
GGSGDDHLH

SEQ ID NO: 16735 - protein, 9 aa, synthetic construct
GGKGQDIFI

SEQ ID NO: 16736 - protein, 9 aa, synthetic construct
GGDGQDVLI

SEQ ID NO: 16737 - protein, 9 aa, synthetic construct
GGTGGDTLL

SEQ ID NO: 16738 - protein, 9 aa, synthetic construct
GGTGGDVFL

SEQ ID NO: 16739 - protein, 9 aa, synthetic construct
GGSGDDFVY

SEQ ID NO: 16740 - protein, 9 aa, synthetic construct
GGTGADVIN

SEQ ID NO: 16741 - protein, 9 aa, synthetic construct
GGTGGDYLD

SEQ ID NO: 16742 - protein, 9 aa, synthetic construct
GGGGNDWLI

SEQ ID NO: 16743 - protein, 9 aa, synthetic construct
GGTGHDDLD

SEQ ID NO: 16744 - protein, 9 aa, synthetic construct
GGSGHDQVY

SEQ ID NO: 16745 - protein, 9 aa, synthetic construct
GGNGADVIL

SEQ ID NO: 16746 - protein, 9 aa, synthetic construct
GGDGNDMIF

SEQ ID NO: 16747 - protein, 9 aa, synthetic construct
GGAGGDSID

SEQ ID NO: 16748 - protein, 9 aa, synthetic construct
GGNGDDFLI

SEQ ID NO: 16749 - protein, 9 aa, synthetic construct
GGEGADYID

SEQ ID NO: 16750 - protein, 9 aa, synthetic construct
GGKGQDSLY

SEQ ID NO: 16751 - protein, 9 aa, synthetic construct
GGTGGDVLR

SEQ ID NO: 16752 - protein, 9 aa, synthetic construct
GGSGDDFLL

SEQ ID NO: 16753 - protein, 9 aa, synthetic construct
GGAGGDSIE

SEQ ID NO: 16754 - protein, 9 aa, synthetic construct
GGNGADVIY

SEQ ID NO: 16755 - protein, 9 aa, synthetic construct
GGSGDDFLR

SEQ ID NO: 16756 - protein, 9 aa, synthetic construct
GGAGGDSIS

SEQ ID NO: 16757 - protein, 9 aa, synthetic construct
GGAGGDSLE

SEQ ID NO: 16758 - protein, 9 aa, synthetic construct
GGDGNDMIW

SEQ ID NO: 16759 - protein, 9 aa, synthetic construct
GGAGGDSLG

SEQ ID NO: 16760 - protein, 9 aa, synthetic construct
GGSGDDHLY

SEQ ID NO: 16761 - protein, 9 aa, synthetic construct
GGKGQDEIY

SEQ ID NO: 16762 - protein, 9 aa, synthetic construct
GGAGGDTMS

SEQ ID NO: 16763 - protein, 9 aa, synthetic construct
GGTGGDTLA

SEQ ID NO: 16764 - protein, 9 aa, synthetic construct
GGIGNDQLD

SEQ ID NO: 16765 - protein, 9 aa, synthetic construct
GGDGNDMLT

SEQ ID NO: 16766 - protein, 9 aa, synthetic construct
GGDGDDLAL

SEQ ID NO: 16767 - protein, 9 aa, synthetic construct
GGAGNDSAI

SEQ ID NO: 16768 - protein, 9 aa, synthetic construct
GGSGDDIYI

SEQ ID NO: 16769 - protein, 9 aa, synthetic construct
GGSGDDIYL

SEQ ID NO: 16770 - protein, 9 aa, synthetic construct
GGSGHDKLI

SEQ ID NO: 16771 - protein, 9 aa, synthetic construct
GGSGHDKLF

SEQ ID NO: 16772 - protein, 9 aa, synthetic construct
GGIGNDQLK

SEQ ID NO: 16773 - protein, 9 aa, synthetic construct
GGIGRDVMD

SEQ ID NO: 16774 - protein, 9 aa, synthetic construct
GGTGGDLLY

SEQ ID NO: 16775 - protein, 9 aa, synthetic construct
GGAGNDRYF

SEQ ID NO: 16776 - protein, 9 aa, synthetic construct
GGTGGDLLD

SEQ ID NO: 16777 - protein, 9 aa, synthetic construct
GGKGNDFID

SEQ ID NO: 16778 - protein, 9 aa, synthetic construct
GGSGDDKLH

SEQ ID NO: 16779 - protein, 9 aa, synthetic construct
GGNGADVLY

SEQ ID NO: 16780 - protein, 9 aa, synthetic construct
GGSGDDKLN

SEQ ID NO: 16781 - protein, 9 aa, synthetic construct
GGSGDDKLR

SEQ ID NO: 16782 - protein, 9 aa, synthetic construct
GGEGDDMLT

SEQ ID NO: 16783 - protein, 9 aa, synthetic construct
GGNGADVLV

SEQ ID NO: 16784 - protein, 9 aa, synthetic construct
GGAGNDSAY

SEQ ID NO: 16785 - protein, 9 aa, synthetic construct
GGDGDDIVN

SEQ ID NO: 16786 - protein, 9 aa, synthetic construct
GGDGNDMLM

SEQ ID NO: 16787 - protein, 9 aa, synthetic construct
GGFGADILV

SEQ ID NO: 16788 - protein, 9 aa, synthetic construct
GGIGNDMLI

SEQ ID NO: 16789 - protein, 9 aa, synthetic construct
GGDGRDRLV

SEQ ID NO: 16790 - protein, 9 aa, synthetic construct
GGTGGDTFV

SEQ ID NO: 16791 - protein, 9 aa, synthetic construct
GGIGNDMLN

SEQ ID NO: 16792 - protein, 9 aa, synthetic construct
GGTGADVLQ

SEQ ID NO: 16793 - protein, 9 aa, synthetic construct
GGAGGDTIA

SEQ ID NO: 16794 - protein, 9 aa, synthetic construct
GGSGDDIIR

SEQ ID NO: 16795 - protein, 9 aa, synthetic construct
GGSGDDIIT

SEQ ID NO: 16796 - protein, 9 aa, synthetic construct
GGTGADVLY

SEQ ID NO: 16797 - protein, 9 aa, synthetic construct
GGDGRDRLQ

SEQ ID NO: 16798 - protein, 9 aa, synthetic construct
GGTGGDSIL

SEQ ID NO: 16799 - protein, 9 aa, synthetic construct
GGTGADVLV

SEQ ID NO: 16800 - protein, 9 aa, synthetic construct
GGIGNDNLD

SEQ ID NO: 16801 - protein, 9 aa, synthetic construct
GGDGRDRLG

SEQ ID NO: 16802 - protein, 9 aa, synthetic construct
GGSGDDILM

SEQ ID NO: 16803 - protein, 9 aa, synthetic construct
GGDGRDRLF

SEQ ID NO: 16804 - protein, 9 aa, synthetic construct
GGAGGDTIS

SEQ ID NO: 16805 - protein, 9 aa, synthetic construct
GGGGADHMV

SEQ ID NO: 16806 - protein, 9 aa, synthetic construct
GGTGNDVVS

SEQ ID NO: 16807 - protein, 9 aa, synthetic construct
GGKGNDILQ

SEQ ID NO: 16808 - protein, 9 aa, synthetic construct
GGTGVDVLR

SEQ ID NO: 16809 - protein, 9 aa, synthetic construct
GGLGDDVLG

SEQ ID NO: 16810 - protein, 9 aa, synthetic construct
GGTGVDVLI

SEQ ID NO: 16811 - protein, 9 aa, synthetic construct
GGIGYDIID

SEQ ID NO: 16812 - protein, 9 aa, synthetic construct
GGQGSDTIR

SEQ ID NO: 16813 - protein, 9 aa, synthetic construct
GGQGSDTLE

SEQ ID NO: 16814 - protein, 9 aa, synthetic construct
GGSGWDTLI

SEQ ID NO: 16815 - protein, 9 aa, synthetic construct
GGQGSDTLL

SEQ ID NO: 16816 - protein, 9 aa, synthetic construct
GGAGMDYLD

SEQ ID NO: 16817 - protein, 9 aa, synthetic construct
GGEGGDRLV

SEQ ID NO: 16818 - protein, 9 aa, synthetic construct
GGTGVDTMI

SEQ ID NO: 16819 - protein, 9 aa, synthetic construct
GGQGSDTLV

SEQ ID NO: 16820 - protein, 9 aa, synthetic construct
GGLGDDVLH

SEQ ID NO: 16821 - protein, 9 aa, synthetic construct
GGIGXDSLN

SEQ ID NO: 16822 - protein, 9 aa, synthetic construct
GGTGVDTLQ

SEQ ID NO: 16823 - protein, 9 aa, synthetic construct
GGNGDDTVK

SEQ ID NO: 16824 - protein, 9 aa, synthetic construct
GGVGDDVAY

SEQ ID NO: 16825 - protein, 9 aa, synthetic construct
GGSGWDTVH

SEQ ID NO: 16826 - protein, 9 aa, synthetic construct
GGAGDDSFI

SEQ ID NO: 16827 - protein, 9 aa, synthetic construct
GGEGGDRLS

SEQ ID NO: 16828 - protein, 9 aa, synthetic construct
GGLGDDVIF

SEQ ID NO: 16829 - protein, 9 aa, synthetic construct
GGLGTDVAR

SEQ ID NO: 16830 - protein, 9 aa, synthetic construct
GGAGMDVLR

SEQ ID NO: 16831 - protein, 9 aa, synthetic construct
GGAGSDDMY

SEQ ID NO: 16832 - protein, 9 aa, synthetic construct
GGDGDDMVI

SEQ ID NO: 16833 - protein, 9 aa, synthetic construct
GGAGSDDLY

SEQ ID NO: 16834 - protein, 9 aa, synthetic construct
GGSGVDILF

SEQ ID NO: 16835 - protein, 9 aa, synthetic construct
GGSGWDQLW

SEQ ID NO: 16836 - protein, 9 aa, synthetic construct
GGNGDDLIN

SEQ ID NO: 16837 - protein, 9 aa, synthetic construct
GGDGDDDVY

SEQ ID NO: 16838 - protein, 9 aa, synthetic construct
GGDGDDTYF

SEQ ID NO: 16839 - protein, 9 aa, synthetic construct
GGQGSDRYI

SEQ ID NO: 16840 - protein, 9 aa, synthetic construct
GGVGDDVAA

SEQ ID NO: 16841 - protein, 9 aa, synthetic construct
GGLGDDLVQ

SEQ ID NO: 16842 - protein, 9 aa, synthetic construct
GGTGVDWMY

SEQ ID NO: 16843 - protein, 9 aa, synthetic construct
GGIGYDRIF

SEQ ID NO: 16844 - protein, 9 aa, synthetic construct
GGQGSDSLF

SEQ ID NO: 16845 - protein, 9 aa, synthetic construct
GGQGSDSLT

SEQ ID NO: 16846 - protein, 9 aa, synthetic construct
GGEGSDTIQ

SEQ ID NO: 16847 - protein, 9 aa, synthetic construct
GGSGNDFLR

SEQ ID NO: 16848 - protein, 9 aa, synthetic construct
GGQGSDTYV

SEQ ID NO: 16849 - protein, 9 aa, synthetic construct
GGGGADRMT

SEQ ID NO: 16850 - protein, 9 aa, synthetic construct
GGAGSDAVH

SEQ ID NO: 16851 - protein, 9 aa, synthetic construct
GGMGSDTIR

SEQ ID NO: 16852 - protein, 9 aa, synthetic construct
GGAGRDYVS

SEQ ID NO: 16853 - protein, 9 aa, synthetic construct
GGTGVDNIT

SEQ ID NO: 16854 - protein, 9 aa, synthetic construct
GGTGVDNID

SEQ ID NO: 16855 - protein, 9 aa, synthetic construct
GGAGDDSMF

SEQ ID NO: 16856 - protein, 9 aa, synthetic construct
GGAGNDAAD

SEQ ID NO: 16857 - protein, 9 aa, synthetic construct
GGGGNDTAT

SEQ ID NO: 16858 - protein, 9 aa, synthetic construct
GGSGNDFIS

SEQ ID NO: 16859 - protein, 9 aa, synthetic construct
GGAGRDYLN

SEQ ID NO: 16860 - protein, 9 aa, synthetic construct
GGAGRDYLI

SEQ ID NO: 16861 - protein, 9 aa, synthetic construct
GGDGSDVIS

SEQ ID NO: 16862 - protein, 9 aa, synthetic construct
GGSGNDFIL

SEQ ID NO: 16863 - protein, 9 aa, synthetic construct
GGAGIDSLR

SEQ ID NO: 16864 - protein, 9 aa, synthetic construct
GGHGNDSLT

SEQ ID NO: 16865 - protein, 9 aa, synthetic construct
GGAGRDYLA

SEQ ID NO: 16866 - protein, 9 aa, synthetic construct
GGQGTDTLY

SEQ ID NO: 16867 - protein, 9 aa, synthetic construct
GGAGRDYIW

SEQ ID NO: 16868 - protein, 9 aa, synthetic construct
GGAGSDAFE

SEQ ID NO: 16869 - protein, 9 aa, synthetic construct
GGIGADIIH

SEQ ID NO: 16870 - protein, 9 aa, synthetic construct
GGAGIDSLV

SEQ ID NO: 16871 - protein, 9 aa, synthetic construct
GGAGMDYLL

SEQ ID NO: 16872 - protein, 9 aa, synthetic construct
GGTGVDTIY

SEQ ID NO: 16873 - protein, 9 aa, synthetic construct
GGAGDDSIG

SEQ ID NO: 16874 - protein, 9 aa, synthetic construct
GGTGVDTIT

SEQ ID NO: 16875 - protein, 9 aa, synthetic construct
GGMGSDSLS

SEQ ID NO: 16876 - protein, 9 aa, synthetic construct
GGTGVDTAV

SEQ ID NO: 16877 - protein, 9 aa, synthetic construct
GGNGDDTVL

SEQ ID NO: 16878 - protein, 9 aa, synthetic construct
GGDGDDTVV

SEQ ID NO: 16879 - protein, 9 aa, synthetic construct
GGAGSDALI

SEQ ID NO: 16880 - protein, 9 aa, synthetic construct
GGTGVDRIN

SEQ ID NO: 16881 - protein, 9 aa, synthetic construct
GGSGNDFLE

SEQ ID NO: 16882 - protein, 9 aa, synthetic construct
GGLGDDLLH

SEQ ID NO: 16883 - protein, 9 aa, synthetic construct
GGAGSDAIS

SEQ ID NO: 16884 - protein, 9 aa, synthetic construct
GGTGVDRMT

SEQ ID NO: 16885 - protein, 9 aa, synthetic construct
GGAGDDSLK

SEQ ID NO: 16886 - protein, 9 aa, synthetic construct
GGMGSDTID

SEQ ID NO: 16887 - protein, 9 aa, synthetic construct
GGQGTDLLQ

SEQ ID NO: 16888 - protein, 9 aa, synthetic construct
GGAGDDRVY

SEQ ID NO: 16889 - protein, 9 aa, synthetic construct
GGAGIDVLF

SEQ ID NO: 16890 - protein, 9 aa, synthetic construct
GGAGIDVLD

SEQ ID NO: 16891 - protein, 9 aa, synthetic construct
GGHGYDILN

SEQ ID NO: 16892 - protein, 9 aa, synthetic construct
GGAGSDFLK

SEQ ID NO: 16893 - protein, 9 aa, synthetic construct
GGVGADDLS

SEQ ID NO: 16894 - protein, 9 aa, synthetic construct
GGDGNDTAY

SEQ ID NO: 16895 - protein, 9 aa, synthetic construct
GGVGDDTMS

SEQ ID NO: 16896 - protein, 9 aa, synthetic construct
GGGGRDEMS

SEQ ID NO: 16897 - protein, 9 aa, synthetic construct
GGVGADALD

SEQ ID NO: 16898 - protein, 9 aa, synthetic construct
GGAGDDRIW

SEQ ID NO: 16899 - protein, 9 aa, synthetic construct
GGGGRDLLD

SEQ ID NO: 16900 - protein, 9 aa, synthetic construct
GGSGNDGLL

SEQ ID NO: 16901 - protein, 9 aa, synthetic construct
GGDGFDTLV

SEQ ID NO: 16902 - protein, 9 aa, synthetic construct
GGDGNDTAT

SEQ ID NO: 16903 - protein, 9 aa, synthetic construct
GGSGNDGLD

SEQ ID NO: 16904 - protein, 9 aa, synthetic construct
GGEGDDVIH

SEQ ID NO: 16905 - protein, 9 aa, synthetic construct
GGFGNDTFS

SEQ ID NO: 16906 - protein, 9 aa, synthetic construct
GGSGNDGIT

SEQ ID NO: 16907 - protein, 9 aa, synthetic construct
GGTGYDTLS

SEQ ID NO: 16908 - protein, 9 aa, synthetic construct
GGSGNDGIR

SEQ ID NO: 16909 - protein, 9 aa, synthetic construct
GGGGADSVA

SEQ ID NO: 16910 - protein, 9 aa, synthetic construct
GGGGHDRLI

SEQ ID NO: 16911 - protein, 9 aa, synthetic construct
GGGGNDFYY

SEQ ID NO: 16912 - protein, 9 aa, synthetic construct
GGHGNDTLE

SEQ ID NO: 16913 - protein, 9 aa, synthetic construct
GGAGSDGLN

SEQ ID NO: 16914 - protein, 9 aa, synthetic construct
GGEGSDTFK

SEQ ID NO: 16915 - protein, 9 aa, synthetic construct
GGAGSDGLD

SEQ ID NO: 16916 - protein, 9 aa, synthetic construct
GGVGADIFV

SEQ ID NO: 16917 - protein, 9 aa, synthetic construct
GGSGNDGVY

SEQ ID NO: 16918 - protein, 9 aa, synthetic construct
GGNGDDLIL

SEQ ID NO: 16919 - protein, 9 aa, synthetic construct
GGAGDDRFD

SEQ ID NO: 16920 - protein, 9 aa, synthetic construct
GGLGDDVIH

SEQ ID NO: 16921 - protein, 9 aa, synthetic construct
GGDGTDLLD

SEQ ID NO: 16922 - protein, 9 aa, synthetic construct
GGGGHDRLF

SEQ ID NO: 16923 - protein, 9 aa, synthetic construct
GGQGRDQLH

SEQ ID NO: 16924 - protein, 9 aa, synthetic construct
GGEGGDRLF

SEQ ID NO: 16925 - protein, 9 aa, synthetic construct
GGVGADFLD

SEQ ID NO: 16926 - protein, 9 aa, synthetic construct
GGGGRDEVY

SEQ ID NO: 16927 - protein, 9 aa, synthetic construct
GGVGADELQ

SEQ ID NO: 16928 - protein, 9 aa, synthetic construct
GGAGSDFLT

SEQ ID NO: 16929 - protein, 9 aa, synthetic construct
GGHGWDTMH

SEQ ID NO: 16930 - protein, 9 aa, synthetic construct
GGQGRDYFV

SEQ ID NO: 16931 - protein, 9 aa, synthetic construct
GGGGNDEMR

SEQ ID NO: 16932 - protein, 9 aa, synthetic construct
GGAGDDRME

SEQ ID NO: 16933 - protein, 9 aa, synthetic construct
GGSGVDIMS

SEQ ID NO: 16934 - protein, 9 aa, synthetic construct
GGGGADSIS

SEQ ID NO: 16935 - protein, 9 aa, synthetic construct
GGLGDDVIS

SEQ ID NO: 16936 - protein, 9 aa, synthetic construct
GGLGDDMLD

SEQ ID NO: 16937 - protein, 9 aa, synthetic construct
GGDGDDLIK

SEQ ID NO: 16938 - protein, 9 aa, synthetic construct
GGLGRDLLH

SEQ ID NO: 16939 - protein, 9 aa, synthetic construct
GGQGSDLLD

SEQ ID NO: 16940 - protein, 9 aa, synthetic construct
GGAGDDRVQ

SEQ ID NO: 16941 - protein, 9 aa, synthetic construct
GGQGSDLLI

SEQ ID NO: 16942 - protein, 9 aa, synthetic construct
GGIGADALY

SEQ ID NO: 16943 - protein, 9 aa, synthetic construct
GGQGSDLLS

SEQ ID NO: 16944 - protein, 9 aa, synthetic construct
GGMGSDILI

SEQ ID NO: 16945 - protein, 9 aa, synthetic construct
GGVGDDTVT

SEQ ID NO: 16946 - protein, 9 aa, synthetic construct
GGAGDDRVT

SEQ ID NO: 16947 - protein, 9 aa, synthetic construct
GGDGDDDVS

SEQ ID NO: 16948 - protein, 9 aa, synthetic construct
GGGGRDELR

SEQ ID NO: 16949 - protein, 9 aa, synthetic construct
GGTGWDNLS

SEQ ID NO: 16950 - protein, 9 aa, synthetic construct
GGLGDDVIQ

SEQ ID NO: 16951 - protein, 9 aa, synthetic construct
GGQGSDIII

SEQ ID NO: 16952 - protein, 9 aa, synthetic construct
GGAGSDELD

SEQ ID NO: 16953 - protein, 9 aa, synthetic construct
GGDGDDDVF

SEQ ID NO: 16954 - protein, 9 aa, synthetic construct
GGGGADSLH

SEQ ID NO: 16955 - protein, 9 aa, synthetic construct
GGQGRDYLE

SEQ ID NO: 16956 - protein, 9 aa, synthetic construct
GGGGNDGIV

SEQ ID NO: 16957 - protein, 9 aa, synthetic construct
GGGGRDELY

SEQ ID NO: 16958 - protein, 9 aa, synthetic construct
GGAGSDFAD

SEQ ID NO: 16959 - protein, 9 aa, synthetic construct
GGMGSDIIT

SEQ ID NO: 16960 - protein, 9 aa, synthetic construct
GGEGDDDIY

SEQ ID NO: 16961 - protein, 9 aa, synthetic construct
GGAGSDELV

SEQ ID NO: 16962 - protein, 9 aa, synthetic construct
GGSGNDFVY

SEQ ID NO: 16963 - protein, 9 aa, synthetic construct
GGQGSDFIS

SEQ ID NO: 16964 - protein, 9 aa, synthetic construct
GGAGMDVLE

SEQ ID NO: 16965 - protein, 9 aa, synthetic construct
GGSGNDLIQ

SEQ ID NO: 16966 - protein, 9 aa, synthetic construct
GGNGKDAIY

SEQ ID NO: 16967 - protein, 9 aa, synthetic construct
GGTGYDLLR

SEQ ID NO: 16968 - protein, 9 aa, synthetic construct
GGAGSDRMA

SEQ ID NO: 16969 - protein, 9 aa, synthetic construct
GGAGMDVLN

SEQ ID NO: 16970 - protein, 9 aa, synthetic construct
GGAGRDYID

SEQ ID NO: 16971 - protein, 9 aa, synthetic construct
GGDGFDIMV

SEQ ID NO: 16972 - protein, 9 aa, synthetic construct
GGAGRDYFR

SEQ ID NO: 16973 - protein, 9 aa, synthetic construct
GGEGNDTMF

SEQ ID NO: 16974 - protein, 9 aa, synthetic construct
GGRGADLLA

SEQ ID NO: 16975 - protein, 9 aa, synthetic construct
GGDGSDTVV

SEQ ID NO: 16976 - protein, 9 aa, synthetic construct
GGRGADLLK

SEQ ID NO: 16977 - protein, 9 aa, synthetic construct
GGLGTDTME

SEQ ID NO: 16978 - protein, 9 aa, synthetic construct
GGFGDDYIS

SEQ ID NO: 16979 - protein, 9 aa, synthetic construct
GGRGADLLR

SEQ ID NO: 16980 - protein, 9 aa, synthetic construct
GGQGHDVVR

SEQ ID NO: 16981 - protein, 9 aa, synthetic construct
GGEGNDTMD

SEQ ID NO: 16982 - protein, 9 aa, synthetic construct
GGDGSDTVT

SEQ ID NO: 16983 - protein, 9 aa, synthetic construct
GGRGADLMD

SEQ ID NO: 16984 - protein, 9 aa, synthetic construct
GGLGDDIIN

SEQ ID NO: 16985 - protein, 9 aa, synthetic construct
GGDGMDTLW

SEQ ID NO: 16986 - protein, 9 aa, synthetic construct
GGEGADRLL

SEQ ID NO: 16987 - protein, 9 aa, synthetic construct
GGEGADVLL

SEQ ID NO: 16988 - protein, 9 aa, synthetic construct
GGAGRDTVA

SEQ ID NO: 16989 - protein, 9 aa, synthetic construct
GGRGADMLR

SEQ ID NO: 16990 - protein, 9 aa, synthetic construct
GGLGDDVML

SEQ ID NO: 16991 - protein, 9 aa, synthetic construct
GGDGGDTIY

SEQ ID NO: 16992 - protein, 9 aa, synthetic construct
GGRGADLIY

SEQ ID NO: 16993 - protein, 9 aa, synthetic construct
GGVGDDWLQ

SEQ ID NO: 16994 - protein, 9 aa, synthetic construct
GGVGDDWLF

SEQ ID NO: 16995 - protein, 9 aa, synthetic construct
GGLGDDILQ

SEQ ID NO: 16996 - protein, 9 aa, synthetic construct
GGTGTDSLS

SEQ ID NO: 16997 - protein, 9 aa, synthetic construct
GGTGTDSLL

SEQ ID NO: 16998 - protein, 9 aa, synthetic construct
GGDGQDILS

SEQ ID NO: 16999 - protein, 9 aa, synthetic construct
GGDGDDTVE

SEQ ID NO: 17000 - protein, 9 aa, synthetic construct
GGQGIDRFV

SEQ ID NO: 17001 - protein, 9 aa, synthetic construct
GGGGADQYA

SEQ ID NO: 17002 - protein, 9 aa, synthetic construct
GGKGADILF

SEQ ID NO: 17003 - protein, 9 aa, synthetic construct
GGTGTDRAV

SEQ ID NO: 17004 - protein, 9 aa, synthetic construct
GGRGADKLT

SEQ ID NO: 17005 - protein, 9 aa, synthetic construct
GGRGADKLV

SEQ ID NO: 17006 - protein, 9 aa, synthetic construct
GGTGTDSFV

SEQ ID NO: 17007 - protein, 9 aa, synthetic construct
GGRGADKMN

SEQ ID NO: 17008 - protein, 9 aa, synthetic construct
GGSGNDEII

SEQ ID NO: 17009 - protein, 9 aa, synthetic construct
GGRGADLFS

SEQ ID NO: 17010 - protein, 9 aa, synthetic construct
GGSGYDRLF

SEQ ID NO: 17011 - protein, 9 aa, synthetic construct
GGFGNDTIS

SEQ ID NO: 17012 - protein, 9 aa, synthetic construct
GGDGQDILV

SEQ ID NO: 17013 - protein, 9 aa, synthetic construct
GGSGNDEIT

SEQ ID NO: 17014 - protein, 9 aa, synthetic construct
GGLGDDIFD

SEQ ID NO: 17015 - protein, 9 aa, synthetic construct
GGTGTDILD

SEQ ID NO: 17016 - protein, 9 aa, synthetic construct
GGRGADRLS

SEQ ID NO: 17017 - protein, 9 aa, synthetic construct
GGTGTDIAS

SEQ ID NO: 17018 - protein, 9 aa, synthetic construct
GGEGSDTYI

SEQ ID NO: 17019 - protein, 9 aa, synthetic construct
GGAGSDNLY

SEQ ID NO: 17020 - protein, 9 aa, synthetic construct
GGDGFDLAS

SEQ ID NO: 17021 - protein, 9 aa, synthetic construct
GGNGIDRIY

SEQ ID NO: 17022 - protein, 9 aa, synthetic construct
GGSGNDDLT

SEQ ID NO: 17023 - protein, 9 aa, synthetic construct
GGAGDDTVR

SEQ ID NO: 17024 - protein, 9 aa, synthetic construct
GGDGFDLFL

SEQ ID NO: 17025 - protein, 9 aa, synthetic construct
GGEGNDTFE

SEQ ID NO: 17026 - protein, 9 aa, synthetic construct
GGTGTDFLD

SEQ ID NO: 17027 - protein, 9 aa, synthetic construct
GGSGYDTLV

SEQ ID NO: 17028 - protein, 9 aa, synthetic construct
GGAGDDTYG

SEQ ID NO: 17029 - protein, 9 aa, synthetic construct
GGTGTDAMA

SEQ ID NO: 17030 - protein, 9 aa, synthetic construct
GGLGDDHIV

SEQ ID NO: 17031 - protein, 9 aa, synthetic construct
GGTGTDALI

SEQ ID NO: 17032 - protein, 9 aa, synthetic construct
GGTGTDILN

SEQ ID NO: 17033 - protein, 9 aa, synthetic construct
GGNGIDRLD

SEQ ID NO: 17034 - protein, 9 aa, synthetic construct
GGRGADRLI

SEQ ID NO: 17035 - protein, 9 aa, synthetic construct
GGAGRDTMD

SEQ ID NO: 17036 - protein, 9 aa, synthetic construct
GGAGRDTMR

SEQ ID NO: 17037 - protein, 9 aa, synthetic construct
GGQGHDTYV

SEQ ID NO: 17038 - protein, 9 aa, synthetic construct
GGGGNDIFD

SEQ ID NO: 17039 - protein, 9 aa, synthetic construct
GGRGADQLA

SEQ ID NO: 17040 - protein, 9 aa, synthetic construct
GGDGMDVFV

SEQ ID NO: 17041 - protein, 9 aa, synthetic construct
GGGGADQLV

SEQ ID NO: 17042 - protein, 9 aa, synthetic construct
GGLGDDVVH

SEQ ID NO: 17043 - protein, 9 aa, synthetic construct
GGLGDDHME

SEQ ID NO: 17044 - protein, 9 aa, synthetic construct
GGIGADQLT

SEQ ID NO: 17045 - protein, 9 aa, synthetic construct
GGAGRDTLW

SEQ ID NO: 17046 - protein, 9 aa, synthetic construct
GGNGKDVLK

SEQ ID NO: 17047 - protein, 9 aa, synthetic construct
GGTGTDKLY

SEQ ID NO: 17048 - protein, 9 aa, synthetic construct
GGTGTDKLT

SEQ ID NO: 17049 - protein, 9 aa, synthetic construct
GGDGDDTMN

SEQ ID NO: 17050 - protein, 9 aa, synthetic construct
GGDGLDNLS

SEQ ID NO: 17051 - protein, 9 aa, synthetic construct
GGMGNDVLD

SEQ ID NO: 17052 - protein, 9 aa, synthetic construct
GGTGTDSMY

SEQ ID NO: 17053 - protein, 9 aa, synthetic construct
GGRGADILT

SEQ ID NO: 17054 - protein, 9 aa, synthetic construct
GGEGDDDAE

SEQ ID NO: 17055 - protein, 9 aa, synthetic construct
GGQGYDLLH

SEQ ID NO: 17056 - protein, 9 aa, synthetic construct
GGSGYDILI

SEQ ID NO: 17057 - protein, 9 aa, synthetic construct
GGTGTDWAT

SEQ ID NO: 17058 - protein, 9 aa, synthetic construct
GGVGDDVLK

SEQ ID NO: 17059 - protein, 9 aa, synthetic construct
GGSGNDLLM

SEQ ID NO: 17060 - protein, 9 aa, synthetic construct
GGAGNDAIG

SEQ ID NO: 17061 - protein, 9 aa, synthetic construct
GGIGVDVLR

SEQ ID NO: 17062 - protein, 9 aa, synthetic construct
GGGGADVLE

SEQ ID NO: 17063 - protein, 9 aa, synthetic construct
GGTGTDVLY

SEQ ID NO: 17064 - protein, 9 aa, synthetic construct
GGLGDDKLD

SEQ ID NO: 17065 - protein, 9 aa, synthetic construct
GGDGDDEIQ

SEQ ID NO: 17066 - protein, 9 aa, synthetic construct
GGQGWDRID

SEQ ID NO: 17067 - protein, 9 aa, synthetic construct
GGQGWDTLI

SEQ ID NO: 17068 - protein, 9 aa, synthetic construct
GGTGTDVLD

SEQ ID NO: 17069 - protein, 9 aa, synthetic construct
GGIGADLIR

SEQ ID NO: 17070 - protein, 9 aa, synthetic construct
GGNGDDTVS

SEQ ID NO: 17071 - protein, 9 aa, synthetic construct
GGDGDDEIR

SEQ ID NO: 17072 - protein, 9 aa, synthetic construct
GGEGSDQLY

SEQ ID NO: 17073 - protein, 9 aa, synthetic construct
GGGGADRIE

SEQ ID NO: 17074 - protein, 9 aa, synthetic construct
GGTGTDWLD

SEQ ID NO: 17075 - protein, 9 aa, synthetic construct
GGDGSDVIF

SEQ ID NO: 17076 - protein, 9 aa, synthetic construct
GGNGDDTVN

SEQ ID NO: 17077 - protein, 9 aa, synthetic construct
GGIGADIMF

SEQ ID NO: 17078 - protein, 9 aa, synthetic construct
GGAGSDSAS

SEQ ID NO: 17079 - protein, 9 aa, synthetic construct
GGAGRDWVN

SEQ ID NO: 17080 - protein, 9 aa, synthetic construct
GGAGDDSVY

SEQ ID NO: 17081 - protein, 9 aa, synthetic construct
GGTGVDELV

SEQ ID NO: 17082 - protein, 9 aa, synthetic construct
GGFGDDTYI

SEQ ID NO: 17083 - protein, 9 aa, synthetic construct
GGEGSDTMS

SEQ ID NO: 17084 - protein, 9 aa, synthetic construct
GGAGNDAFA

SEQ ID NO: 17085 - protein, 9 aa, synthetic construct
GGAGNDAIA

SEQ ID NO: 17086 - protein, 9 aa, synthetic construct
GGGGFDSYY

SEQ ID NO: 17087 - protein, 9 aa, synthetic construct
GGKGHDRLD

SEQ ID NO: 17088 - protein, 9 aa, synthetic construct
GGDGNDTAE

SEQ ID NO: 17089 - protein, 9 aa, synthetic construct
GGDGDDTVI

SEQ ID NO: 17090 - protein, 9 aa, synthetic construct
GGFGDDWID

SEQ ID NO: 17091 - protein, 9 aa, synthetic construct
GGAGQDTVN

SEQ ID NO: 17092 - protein, 9 aa, synthetic construct
GGGGADRIF

SEQ ID NO: 17093 - protein, 9 aa, synthetic construct
GGQGIDYID

SEQ ID NO: 17094 - protein, 9 aa, synthetic construct
GGTGTDTVV

SEQ ID NO: 17095 - protein, 9 aa, synthetic construct
GGQGIDSLF

SEQ ID NO: 17096 - protein, 9 aa, synthetic construct
GGIGADLIY

SEQ ID NO: 17097 - protein, 9 aa, synthetic construct
GGDGQDILI

SEQ ID NO: 17098 - protein, 9 aa, synthetic construct
GGLGRDNYY

SEQ ID NO: 17099 - protein, 9 aa, synthetic construct
GGTGTDTLF

SEQ ID NO: 17100 - protein, 9 aa, synthetic construct
GGRGADELR

SEQ ID NO: 17101 - protein, 9 aa, synthetic construct
GGAGRDVIA

SEQ ID NO: 17102 - protein, 9 aa, synthetic construct
GGGGNDIFA

SEQ ID NO: 17103 - protein, 9 aa, synthetic construct
GGAGDDTFS

SEQ ID NO: 17104 - protein, 9 aa, synthetic construct
GGRGADFLD

SEQ ID NO: 17105 - protein, 9 aa, synthetic construct
GGIGVDTLN

SEQ ID NO: 17106 - protein, 9 aa, synthetic construct
GGTGTDTIT

SEQ ID NO: 17107 - protein, 9 aa, synthetic construct
GGNGIDSLY

SEQ ID NO: 17108 - protein, 9 aa, synthetic construct
GGRGADGLR

SEQ ID NO: 17109 - protein, 9 aa, synthetic construct
GGTGTDTID

SEQ ID NO: 17110 - protein, 9 aa, synthetic construct
GGEGDDVIA

SEQ ID NO: 17111 - protein, 9 aa, synthetic construct
GGGGADRFA

SEQ ID NO: 17112 - protein, 9 aa, synthetic construct
GGQGIDTAI

SEQ ID NO: 17113 - protein, 9 aa, synthetic construct
GGTGTDTAF

SEQ ID NO: 17114 - protein, 9 aa, synthetic construct
GGRGADDLR

SEQ ID NO: 17115 - protein, 9 aa, synthetic construct
GGDGQDILF

SEQ ID NO: 17116 - protein, 9 aa, synthetic construct
GGNGIDTAW

SEQ ID NO: 17117 - protein, 9 aa, synthetic construct
GGSGNDELQ

SEQ ID NO: 17118 - protein, 9 aa, synthetic construct
GGAGRDVLG

SEQ ID NO: 17119 - protein, 9 aa, synthetic construct
GGTGTDTMY

SEQ ID NO: 17120 - protein, 9 aa, synthetic construct
GGAGIDSAY

SEQ ID NO: 17121 - protein, 9 aa, synthetic construct
GGTGTDTMV

SEQ ID NO: 17122 - protein, 9 aa, synthetic construct
GGDGTDLLY

SEQ ID NO: 17123 - protein, 9 aa, synthetic construct
GGRGADALF

SEQ ID NO: 17124 - protein, 9 aa, synthetic construct
GGAGRDVLA

SEQ ID NO: 17125 - protein, 9 aa, synthetic construct
GGAGRDVIV

SEQ ID NO: 17126 - protein, 9 aa, synthetic construct
GGTGTDTMI

SEQ ID NO: 17127 - protein, 9 aa, synthetic construct
GGRGADDFS

SEQ ID NO: 17128 - protein, 9 aa, synthetic construct
GGAGDDTFN

SEQ ID NO: 17129 - protein, 9 aa, synthetic construct
GGIGADLLD

SEQ ID NO: 17130 - protein, 9 aa, synthetic construct
GGVGDDVYE

SEQ ID NO: 17131 - protein, 9 aa, synthetic construct
GGAGSDSIS

SEQ ID NO: 17132 - protein, 9 aa, synthetic construct
GGAGRDVIN

SEQ ID NO: 17133 - protein, 9 aa, synthetic construct
GGKGADILD

SEQ ID NO: 17134 - protein, 9 aa, synthetic construct
GGGGADTFH

SEQ ID NO: 17135 - protein, 9 aa, synthetic construct
GGAGSDGLY

SEQ ID NO: 17136 - protein, 9 aa, synthetic construct
GGLGTDTLK

SEQ ID NO: 17137 - protein, 9 aa, synthetic construct
GGQGNDEIY

SEQ ID NO: 17138 - protein, 9 aa, synthetic construct
GGDGDDDLA

SEQ ID NO: 17139 - protein, 9 aa, synthetic construct
GGLGDDTVR

SEQ ID NO: 17140 - protein, 9 aa, synthetic construct
GGSGVDSIS

SEQ ID NO: 17141 - protein, 9 aa, synthetic construct
GGSGVDSLF

SEQ ID NO: 17142 - protein, 9 aa, synthetic construct
GGGGRDKLN

SEQ ID NO: 17143 - protein, 9 aa, synthetic construct
GGSGVDSLN

SEQ ID NO: 17144 - protein, 9 aa, synthetic construct
GGDGTDIIN

SEQ ID NO: 17145 - protein, 9 aa, synthetic construct
GGSGNDIMI

SEQ ID NO: 17146 - protein, 9 aa, synthetic construct
GGQGNDRLM

SEQ ID NO: 17147 - protein, 9 aa, synthetic construct
GGSGNDIMF

SEQ ID NO: 17148 - protein, 9 aa, synthetic construct
GGAGDDNIG

SEQ ID NO: 17149 - protein, 9 aa, synthetic construct
GGQGNDRLT

SEQ ID NO: 17150 - protein, 9 aa, synthetic construct
GGDGDDVIQ

SEQ ID NO: 17151 - protein, 9 aa, synthetic construct
GGQGNDRLY

SEQ ID NO: 17152 - protein, 9 aa, synthetic construct
GGFGNDSLQ

SEQ ID NO: 17153 - protein, 9 aa, synthetic construct
GGKGGDSLI

SEQ ID NO: 17154 - protein, 9 aa, synthetic construct
GGQGNDRYI

SEQ ID NO: 17155 - protein, 9 aa, synthetic construct
GGQGNDQMR

SEQ ID NO: 17156 - protein, 9 aa, synthetic construct
GGVGDDDLY

SEQ ID NO: 17157 - protein, 9 aa, synthetic construct
GGSGVDYLN

SEQ ID NO: 17158 - protein, 9 aa, synthetic construct
GGVGDDRID

SEQ ID NO: 17159 - protein, 9 aa, synthetic construct
GGSGNDIVG

SEQ ID NO: 17160 - protein, 9 aa, synthetic construct
GGQGNDQFA

SEQ ID NO: 17161 - protein, 9 aa, synthetic construct
GGEGSDRMM

SEQ ID NO: 17162 - protein, 9 aa, synthetic construct
GGQGNDQIF

SEQ ID NO: 17163 - protein, 9 aa, synthetic construct
GGGGRDLIR

SEQ ID NO: 17164 - protein, 9 aa, synthetic construct
GGEGDDDLT

SEQ ID NO: 17165 - protein, 9 aa, synthetic construct
GGVGDDRFV

SEQ ID NO: 17166 - protein, 9 aa, synthetic construct
GGVGDDELY

SEQ ID NO: 17167 - protein, 9 aa, synthetic construct
GGAGDDMVL

SEQ ID NO: 17168 - protein, 9 aa, synthetic construct
GGDGLDTIN

SEQ ID NO: 17169 - protein, 9 aa, synthetic construct
GGDGLDTIS

SEQ ID NO: 17170 - protein, 9 aa, synthetic construct
GGAGDDMVQ

SEQ ID NO: 17171 - protein, 9 aa, synthetic construct
GGVGDDEIH

SEQ ID NO: 17172 - protein, 9 aa, synthetic construct
GGAGDDMVY

SEQ ID NO: 17173 - protein, 9 aa, synthetic construct
GGLGDDTVQ

SEQ ID NO: 17174 - protein, 9 aa, synthetic construct
GGQGNDQLN

SEQ ID NO: 17175 - protein, 9 aa, synthetic construct
GGQGNDELG

SEQ ID NO: 17176 - protein, 9 aa, synthetic construct
GGEGGDLFR

SEQ ID NO: 17177 - protein, 9 aa, synthetic construct
GGLGDDTVT

SEQ ID NO: 17178 - protein, 9 aa, synthetic construct
GGQGNDSAS

SEQ ID NO: 17179 - protein, 9 aa, synthetic construct
GGAGDDNLA

SEQ ID NO: 17180 - protein, 9 aa, synthetic construct
GGQGNDSML

SEQ ID NO: 17181 - protein, 9 aa, synthetic construct
GGQGNDSMT

SEQ ID NO: 17182 - protein, 9 aa, synthetic construct
GGDGLDRLS

SEQ ID NO: 17183 - protein, 9 aa, synthetic construct
GGAGSDLIQ

SEQ ID NO: 17184 - protein, 9 aa, synthetic construct
GGLGDDSLG

SEQ ID NO: 17185 - protein, 9 aa, synthetic construct
GGAGSDLIN

SEQ ID NO: 17186 - protein, 9 aa, synthetic construct
GGSGVDTIF

SEQ ID NO: 17187 - protein, 9 aa, synthetic construct
GGSGVDTII

SEQ ID NO: 17188 - protein, 9 aa, synthetic construct
GGVGADVLM

SEQ ID NO: 17189 - protein, 9 aa, synthetic construct
GGSGVDTIL

SEQ ID NO: 17190 - protein, 9 aa, synthetic construct
GGDGTDFLL

SEQ ID NO: 17191 - protein, 9 aa, synthetic construct
GGSGVDTLD

SEQ ID NO: 17192 - protein, 9 aa, synthetic construct
GGNGKDRLY

SEQ ID NO: 17193 - protein, 9 aa, synthetic construct
GGLGDDSIY

SEQ ID NO: 17194 - protein, 9 aa, synthetic construct
GGVGDDRLL

SEQ ID NO: 17195 - protein, 9 aa, synthetic construct
GGQGNDDIR

SEQ ID NO: 17196 - protein, 9 aa, synthetic construct
GGVGADTYL

SEQ ID NO: 17197 - protein, 9 aa, synthetic construct
GGAGIDTIS

SEQ ID NO: 17198 - protein, 9 aa, synthetic construct
GGSGNDLAF

SEQ ID NO: 17199 - protein, 9 aa, synthetic construct
GGVGDDRLA

SEQ ID NO: 17200 - protein, 9 aa, synthetic construct
GGDGTDHLD

SEQ ID NO: 17201 - protein, 9 aa, synthetic construct
GGKGADELY

SEQ ID NO: 17202 - protein, 9 aa, synthetic construct
GGHGQDQLW

SEQ ID NO: 17203 - protein, 9 aa, synthetic construct
GGEGSDSLE

SEQ ID NO: 17204 - protein, 9 aa, synthetic construct
GGGGNDFID

SEQ ID NO: 17205 - protein, 9 aa, synthetic construct
GGKGADGIS

SEQ ID NO: 17206 - protein, 9 aa, synthetic construct
GGAGSDLLF

SEQ ID NO: 17207 - protein, 9 aa, synthetic construct
GGEGSDSLF

SEQ ID NO: 17208 - protein, 9 aa, synthetic construct
GGAGIDTIW

SEQ ID NO: 17209 - protein, 9 aa, synthetic construct
GGVGADVMI

SEQ ID NO: 17210 - protein, 9 aa, synthetic construct
GGAGIDTYS

SEQ ID NO: 17211 - protein, 9 aa, synthetic construct
GGEGSDSLI

SEQ ID NO: 17212 - protein, 9 aa, synthetic construct
GGAGDDNLN

SEQ ID NO: 17213 - protein, 9 aa, synthetic construct
GGEGADTYV

SEQ ID NO: 17214 - protein, 9 aa, synthetic construct
GGEGADQLT

SEQ ID NO: 17215 - protein, 9 aa, synthetic construct
GGDGTDGLR

SEQ ID NO: 17216 - protein, 9 aa, synthetic construct
GGLGDDSLN

SEQ ID NO: 17217 - protein, 9 aa, synthetic construct
GGGGNDFLF

SEQ ID NO: 17218 - protein, 9 aa, synthetic construct
GGGGNDFLD

SEQ ID NO: 17219 - protein, 9 aa, synthetic construct
GGLGDDSVY

SEQ ID NO: 17220 - protein, 9 aa, synthetic construct
GGLGDDTVD

SEQ ID NO: 17221 - protein, 9 aa, synthetic construct
GGVGDDLLQ

SEQ ID NO: 17222 - protein, 9 aa, synthetic construct
GGLGDDTMI

SEQ ID NO: 17223 - protein, 9 aa, synthetic construct
GGSGNDKLK

SEQ ID NO: 17224 - protein, 9 aa, synthetic construct
GGAGDDLYT

SEQ ID NO: 17225 - protein, 9 aa, synthetic construct
GGEGADQLF

SEQ ID NO: 17226 - protein, 9 aa, synthetic construct
GGQGNDIVA

SEQ ID NO: 17227 - protein, 9 aa, synthetic construct
GGVGDDQLD

SEQ ID NO: 17228 - protein, 9 aa, synthetic construct
GGQGNDIYM

SEQ ID NO: 17229 - protein, 9 aa, synthetic construct
GGQGNDIYY

SEQ ID NO: 17230 - protein, 9 aa, synthetic construct
GGLGDDTIV

SEQ ID NO: 17231 - protein, 9 aa, synthetic construct
GGAGDDLMW

SEQ ID NO: 17232 - protein, 9 aa, synthetic construct
GGQGNDKIY

SEQ ID NO: 17233 - protein, 9 aa, synthetic construct
GGLGDDTMT

SEQ ID NO: 17234 - protein, 9 aa, synthetic construct
GGFGDDVMS

SEQ ID NO: 17235 - protein, 9 aa, synthetic construct
GGVGDDLIF

SEQ ID NO: 17236 - protein, 9 aa, synthetic construct
GGEGADQLH

SEQ ID NO: 17237 - protein, 9 aa, synthetic construct
GGLGDDTIR

SEQ ID NO: 17238 - protein, 9 aa, synthetic construct
GGEGGDLLK

SEQ ID NO: 17239 - protein, 9 aa, synthetic construct
GGMGPDRLF

SEQ ID NO: 17240 - protein, 9 aa, synthetic construct
GGSGNDKLL

SEQ ID NO: 17241 - protein, 9 aa, synthetic construct
GGQGNDIIY

SEQ ID NO: 17242 - protein, 9 aa, synthetic construct
GGGGIDRLY

SEQ ID NO: 17243 - protein, 9 aa, synthetic construct
GGAGDDLVE

SEQ ID NO: 17244 - protein, 9 aa, synthetic construct
GGQGNDGLS

SEQ ID NO: 17245 - protein, 9 aa, synthetic construct
GGEGSDRID

SEQ ID NO: 17246 - protein, 9 aa, synthetic construct
GGQGNDIID

SEQ ID NO: 17247 - protein, 9 aa, synthetic construct
GGAGIDTVA

SEQ ID NO: 17248 - protein, 9 aa, synthetic construct
GGSGVDNLY

SEQ ID NO: 17249 - protein, 9 aa, synthetic construct
GGAGDDLVV

SEQ ID NO: 17250 - protein, 9 aa, synthetic construct
GGEGDDDVN

SEQ ID NO: 17251 - protein, 9 aa, synthetic construct
GGAGDDLVY

SEQ ID NO: 17252 - protein, 9 aa, synthetic construct
GGAGSDNIY

SEQ ID NO: 17253 - protein, 9 aa, synthetic construct
GGVGDDLVL

SEQ ID NO: 17254 - protein, 9 aa, synthetic construct
GGSGNDKLQ

SEQ ID NO: 17255 - protein, 9 aa, synthetic construct
GGAGDDLYA

SEQ ID NO: 17256 - protein, 9 aa, synthetic construct
GGEGSDRLD

SEQ ID NO: 17257 - protein, 9 aa, synthetic construct
GGSGNDKLN

SEQ ID NO: 17258 - protein, 9 aa, synthetic construct
GGHGNDVLG

SEQ ID NO: 17259 - protein, 9 aa, synthetic construct
GGQGNDLIA

SEQ ID NO: 17260 - protein, 9 aa, synthetic construct
GGNGKDTFI

SEQ ID NO: 17261 - protein, 9 aa, synthetic construct
GGVGDDKYY

SEQ ID NO: 17262 - protein, 9 aa, synthetic construct
GGFGNDSIL

SEQ ID NO: 17263 - protein, 9 aa, synthetic construct
GGLGDDTFK

SEQ ID NO: 17264 - protein, 9 aa, synthetic construct
GGLGDDTFI

SEQ ID NO: 17265 - protein, 9 aa, synthetic construct
GGSGNDKAE

SEQ ID NO: 17266 - protein, 9 aa, synthetic construct
GGGGNDFIS

SEQ ID NO: 17267 - protein, 9 aa, synthetic construct
GGDGDDDIR

SEQ ID NO: 17268 - protein, 9 aa, synthetic construct
GGDGLDSLY

SEQ ID NO: 17269 - protein, 9 aa, synthetic construct
GGGGIDRLH

SEQ ID NO: 17270 - protein, 9 aa, synthetic construct
GGQGNDMLL

SEQ ID NO: 17271 - protein, 9 aa, synthetic construct
GGHGNDYLF

SEQ ID NO: 17272 - protein, 9 aa, synthetic construct
GGVGDDIII

SEQ ID NO: 17273 - protein, 9 aa, synthetic construct
GGDGFDTVT

SEQ ID NO: 17274 - protein, 9 aa, synthetic construct
GGDGLDTAS

SEQ ID NO: 17275 - protein, 9 aa, synthetic construct
GGSGVDRMT

SEQ ID NO: 17276 - protein, 9 aa, synthetic construct
GGQGNDNLA

SEQ ID NO: 17277 - protein, 9 aa, synthetic construct
GGDGFDFVS

SEQ ID NO: 17278 - protein, 9 aa, synthetic construct
GGVGDDFLM

SEQ ID NO: 17279 - protein, 9 aa, synthetic construct
GGSGVDRLS

SEQ ID NO: 17280 - protein, 9 aa, synthetic construct
GGAGIDTMD

SEQ ID NO: 17281 - protein, 9 aa, synthetic construct
GGGGRDKVF

SEQ ID NO: 17282 - protein, 9 aa, synthetic construct
GGSGNDKLE

SEQ ID NO: 17283 - protein, 9 aa, synthetic construct
GGGGFDRIN

SEQ ID NO: 17284 - protein, 9 aa, synthetic construct
GGQGNDFIG

SEQ ID NO: 17285 - protein, 9 aa, synthetic construct
GGLGDDTVE

SEQ ID NO: 17286 - protein, 9 aa, synthetic construct
GGEGDDLLR

SEQ ID NO: 17287 - protein, 9 aa, synthetic construct
GGAGSDMLR

SEQ ID NO: 17288 - protein, 9 aa, synthetic construct
GGAGDDMID

SEQ ID NO: 17289 - protein, 9 aa, synthetic construct
GGGGRDLFE

SEQ ID NO: 17290 - protein, 9 aa, synthetic construct
GGEGSDRLI

SEQ ID NO: 17291 - protein, 9 aa, synthetic construct
GGSGVDQMT

SEQ ID NO: 17292 - protein, 9 aa, synthetic construct
GGSGNDKLD

SEQ ID NO: 17293 - protein, 9 aa, synthetic construct
GGVGDDKLD

SEQ ID NO: 17294 - protein, 9 aa, synthetic construct
GGAGDDMIS

SEQ ID NO: 17295 - protein, 9 aa, synthetic construct
GGVGDDIYY

SEQ ID NO: 17296 - protein, 9 aa, synthetic construct
GGVGDDIYV

SEQ ID NO: 17297 - protein, 9 aa, synthetic construct
GGDGTDIVI

SEQ ID NO: 17298 - protein, 9 aa, synthetic construct
GGVGDDIVS

SEQ ID NO: 17299 - protein, 9 aa, synthetic construct
GGGGNDSVN

SEQ ID NO: 17300 - protein, 9 aa, synthetic construct
GGGGNDSVS

SEQ ID NO: 17301 - protein, 9 aa, synthetic construct
GGLGDDSIT

SEQ ID NO: 17302 - protein, 9 aa, synthetic construct
GGKGGDVLR

SEQ ID NO: 17303 - protein, 9 aa, synthetic construct
GGAGMDTLN

SEQ ID NO: 17304 - protein, 9 aa, synthetic construct
GGDGGDTFR

SEQ ID NO: 17305 - protein, 9 aa, synthetic construct
GGEGSDSYY

SEQ ID NO: 17306 - protein, 9 aa, synthetic construct
GGVGADLLT

SEQ ID NO: 17307 - protein, 9 aa, synthetic construct
GGEGSDTAD

SEQ ID NO: 17308 - protein, 9 aa, synthetic construct
GGQGQDKIH

SEQ ID NO: 17309 - protein, 9 aa, synthetic construct
GGQGQDKLI

SEQ ID NO: 17310 - protein, 9 aa, synthetic construct
GGSGNDHLT

SEQ ID NO: 17311 - protein, 9 aa, synthetic construct
GGQGQDLIY

SEQ ID NO: 17312 - protein, 9 aa, synthetic construct
GGAGDDQML

SEQ ID NO: 17313 - protein, 9 aa, synthetic construct
GGQGQDLLE

SEQ ID NO: 17314 - protein, 9 aa, synthetic construct
GGVGADLLK

SEQ ID NO: 17315 - protein, 9 aa, synthetic construct
GGEGDDEAS

SEQ ID NO: 17316 - protein, 9 aa, synthetic construct
GGAGDDQMR

SEQ ID NO: 17317 - protein, 9 aa, synthetic construct
GGLGTDYIY

SEQ ID NO: 17318 - protein, 9 aa, synthetic construct
GGFGDDVYI

SEQ ID NO: 17319 - protein, 9 aa, synthetic construct
GGFGDDVIF

SEQ ID NO: 17320 - protein, 9 aa, synthetic construct
GGLGDDVFK

SEQ ID NO: 17321 - protein, 9 aa, synthetic construct
GGDGLDRLE

SEQ ID NO: 17322 - protein, 9 aa, synthetic construct
GGHGSDVLR

SEQ ID NO: 17323 - protein, 9 aa, synthetic construct
GGSGVDVAS

SEQ ID NO: 17324 - protein, 9 aa, synthetic construct
GGLGDDRMT

SEQ ID NO: 17325 - protein, 9 aa, synthetic construct
GGHGSDTIE

SEQ ID NO: 17326 - protein, 9 aa, synthetic construct
GGAGSDRII

SEQ ID NO: 17327 - protein, 9 aa, synthetic construct
GGAGSDIVW

SEQ ID NO: 17328 - protein, 9 aa, synthetic construct
GGMGRDTLE

SEQ ID NO: 17329 - protein, 9 aa, synthetic construct
GGSGNDHVD

SEQ ID NO: 17330 - protein, 9 aa, synthetic construct
GGDGDDVFT

SEQ ID NO: 17331 - protein, 9 aa, synthetic construct
GGDGSDYME

SEQ ID NO: 17332 - protein, 9 aa, synthetic construct
GGEGSDSVT

SEQ ID NO: 17333 - protein, 9 aa, synthetic construct
GGVGADMLA

SEQ ID NO: 17334 - protein, 9 aa, synthetic construct
GGDGDDDLN

SEQ ID NO: 17335 - protein, 9 aa, synthetic construct
GGGGNDSYY

SEQ ID NO: 17336 - protein, 9 aa, synthetic construct
GGGGADTIE

SEQ ID NO: 17337 - protein, 9 aa, synthetic construct
GGQGQDALL

SEQ ID NO: 17338 - protein, 9 aa, synthetic construct
GGAGSDILY

SEQ ID NO: 17339 - protein, 9 aa, synthetic construct
GGVGADLMN

SEQ ID NO: 17340 - protein, 9 aa, synthetic construct
GGGGADTIA

SEQ ID NO: 17341 - protein, 9 aa, synthetic construct
GGNGDDKLG

SEQ ID NO: 17342 - protein, 9 aa, synthetic construct
GGAGSDIYL

SEQ ID NO: 17343 - protein, 9 aa, synthetic construct
GGQGLDTFV

SEQ ID NO: 17344 - protein, 9 aa, synthetic construct
GGGGNDFVN

SEQ ID NO: 17345 - protein, 9 aa, synthetic construct
GGDGNDTFK

SEQ ID NO: 17346 - protein, 9 aa, synthetic construct
GGVGADILT

SEQ ID NO: 17347 - protein, 9 aa, synthetic construct
GGDGDDDLT

SEQ ID NO: 17348 - protein, 9 aa, synthetic construct
GGSGNDHIF

SEQ ID NO: 17349 - protein, 9 aa, synthetic construct
GGNGDDKLF

SEQ ID NO: 17350 - protein, 9 aa, synthetic construct
GGEGNDELR

SEQ ID NO: 17351 - protein, 9 aa, synthetic construct
GGDGNDTFH

SEQ ID NO: 17352 - protein, 9 aa, synthetic construct
GGAGSDHLT

SEQ ID NO: 17353 - protein, 9 aa, synthetic construct
GGAGSDHLS

SEQ ID NO: 17354 - protein, 9 aa, synthetic construct
GGVGADILL

SEQ ID NO: 17355 - protein, 9 aa, synthetic construct
GGAGSDHLF

SEQ ID NO: 17356 - protein, 9 aa, synthetic construct
GGQGRDELR

SEQ ID NO: 17357 - protein, 9 aa, synthetic construct
GGAGSDHLD

SEQ ID NO: 17358 - protein, 9 aa, synthetic construct
GGAGMDRLL

SEQ ID NO: 17359 - protein, 9 aa, synthetic construct
GGKGHDALT

SEQ ID NO: 17360 - protein, 9 aa, synthetic construct
GGNGKDILF

SEQ ID NO: 17361 - protein, 9 aa, synthetic construct
GGMGRDVLR

SEQ ID NO: 17362 - protein, 9 aa, synthetic construct
GGFGDDVYV

SEQ ID NO: 17363 - protein, 9 aa, synthetic construct
GGLGDDRAD

SEQ ID NO: 17364 - protein, 9 aa, synthetic construct
GGSGNDHLA

SEQ ID NO: 17365 - protein, 9 aa, synthetic construct
GGAGSDIIL

SEQ ID NO: 17366 - protein, 9 aa, synthetic construct
GGQGQDSIS

SEQ ID NO: 17367 - protein, 9 aa, synthetic construct
GGAGDDLLC

SEQ ID NO: 17368 - protein, 9 aa, synthetic construct
GGLGDDRIH

SEQ ID NO: 17369 - protein, 9 aa, synthetic construct
GGDGSDYLI

SEQ ID NO: 17370 - protein, 9 aa, synthetic construct
GGLGDDRIF

SEQ ID NO: 17371 - protein, 9 aa, synthetic construct
GGSGNDHLE

SEQ ID NO: 17372 - protein, 9 aa, synthetic construct
GGAGIDTAK

SEQ ID NO: 17373 - protein, 9 aa, synthetic construct
GGHGNDTLR

SEQ ID NO: 17374 - protein, 9 aa, synthetic construct
GGQGQDTLF

SEQ ID NO: 17375 - protein, 9 aa, synthetic construct
GGGGNDFMN

SEQ ID NO: 17376 - protein, 9 aa, synthetic construct
GGVGADKLY

SEQ ID NO: 17377 - protein, 9 aa, synthetic construct
GGMGNDVYV

SEQ ID NO: 17378 - protein, 9 aa, synthetic construct
GGVGADKLF

SEQ ID NO: 17379 - protein, 9 aa, synthetic construct
GGAGDDQVN

SEQ ID NO: 17380 - protein, 9 aa, synthetic construct
GGVGADKFL

SEQ ID NO: 17381 - protein, 9 aa, synthetic construct
GGAGDDQLM

SEQ ID NO: 17382 - protein, 9 aa, synthetic construct
GGDGLDRLF

SEQ ID NO: 17383 - protein, 9 aa, synthetic construct
GGFGDDVLA

SEQ ID NO: 17384 - protein, 9 aa, synthetic construct
GGAGIDTFI

SEQ ID NO: 17385 - protein, 9 aa, synthetic construct
GGQGNDTVD

SEQ ID NO: 17386 - protein, 9 aa, synthetic construct
GGQGNDTVF

SEQ ID NO: 17387 - protein, 9 aa, synthetic construct
GGVGDDSIT

SEQ ID NO: 17388 - protein, 9 aa, synthetic construct
GGQGNDTVR

SEQ ID NO: 17389 - protein, 9 aa, synthetic construct
GGQGNDTVS

SEQ ID NO: 17390 - protein, 9 aa, synthetic construct
GGSGNDIIE

SEQ ID NO: 17391 - protein, 9 aa, synthetic construct
GGVGADSMA

SEQ ID NO: 17392 - protein, 9 aa, synthetic construct
GGVGADSLY

SEQ ID NO: 17393 - protein, 9 aa, synthetic construct
GGAGSDQMF

SEQ ID NO: 17394 - protein, 9 aa, synthetic construct
GGHGSDLIY

SEQ ID NO: 17395 - protein, 9 aa, synthetic construct
GGGGNDFLM

SEQ ID NO: 17396 - protein, 9 aa, synthetic construct
GGVGADSLR

SEQ ID NO: 17397 - protein, 9 aa, synthetic construct
GGQGNDVAF

SEQ ID NO: 17398 - protein, 9 aa, synthetic construct
GGFGNDSLV

SEQ ID NO: 17399 - protein, 9 aa, synthetic construct
GGEGSDSVL

SEQ ID NO: 17400 - protein, 9 aa, synthetic construct
GGAGSDKLR

SEQ ID NO: 17401 - protein, 9 aa, synthetic construct
GGLGDDTYM

SEQ ID NO: 17402 - protein, 9 aa, synthetic construct
GGVGADSMT

SEQ ID NO: 17403 - protein, 9 aa, synthetic construct
GGAGSDQLY

SEQ ID NO: 17404 - protein, 9 aa, synthetic construct
GGHGSDIFN

SEQ ID NO: 17405 - protein, 9 aa, synthetic construct
GGDGQDELY

SEQ ID NO: 17406 - protein, 9 aa, synthetic construct
GGQGNDTIV

SEQ ID NO: 17407 - protein, 9 aa, synthetic construct
GGGGRDILF

SEQ ID NO: 17408 - protein, 9 aa, synthetic construct
GGVGADTMQ

SEQ ID NO: 17409 - protein, 9 aa, synthetic construct
GGAGDDLMI

SEQ ID NO: 17410 - protein, 9 aa, synthetic construct
GGVGADTMM

SEQ ID NO: 17411 - protein, 9 aa, synthetic construct
GGQGNDDIK

SEQ ID NO: 17412 - protein, 9 aa, synthetic construct
GGVGADTMA

SEQ ID NO: 17413 - protein, 9 aa, synthetic construct
GGHGRDVLF

SEQ ID NO: 17414 - protein, 9 aa, synthetic construct
GGGGRDILA

SEQ ID NO: 17415 - protein, 9 aa, synthetic construct
GGMGRDQLY

SEQ ID NO: 17416 - protein, 9 aa, synthetic construct
GGAGDDLMF

SEQ ID NO: 17417 - protein, 9 aa, synthetic construct
GGVGDDRLY

SEQ ID NO: 17418 - protein, 9 aa, synthetic construct
GGVGADTIR

SEQ ID NO: 17419 - protein, 9 aa, synthetic construct
GGHGSDDID

SEQ ID NO: 17420 - protein, 9 aa, synthetic construct
GGQGNDTMA

SEQ ID NO: 17421 - protein, 9 aa, synthetic construct
GGAGSDKYY

SEQ ID NO: 17422 - protein, 9 aa, synthetic construct
GGVGADSFR

SEQ ID NO: 17423 - protein, 9 aa, synthetic construct
GGQGNDVIE

SEQ ID NO: 17424 - protein, 9 aa, synthetic construct
GGAGDDQLK

SEQ ID NO: 17425 - protein, 9 aa, synthetic construct
GGDGDDDIG

SEQ ID NO: 17426 - protein, 9 aa, synthetic construct
GGAGSDKIY

SEQ ID NO: 17427 - protein, 9 aa, synthetic construct
GGGGFDRLF

SEQ ID NO: 17428 - protein, 9 aa, synthetic construct
GGQGMDWLN

SEQ ID NO: 17429 - protein, 9 aa, synthetic construct
GGVGADQMA

SEQ ID NO: 17430 - protein, 9 aa, synthetic construct
GGVGADQLY

SEQ ID NO: 17431 - protein, 9 aa, synthetic construct
GGVGADQLV

SEQ ID NO: 17432 - protein, 9 aa, synthetic construct
GGDGNDTFY

SEQ ID NO: 17433 - protein, 9 aa, synthetic construct
GGAGSDRFI

SEQ ID NO: 17434 - protein, 9 aa, synthetic construct
GGQGNDWLA

SEQ ID NO: 17435 - protein, 9 aa, synthetic construct
GGLGRDKLV

SEQ ID NO: 17436 - protein, 9 aa, synthetic construct
GGAGSDRFT

SEQ ID NO: 17437 - protein, 9 aa, synthetic construct
GGVGADQLL

SEQ ID NO: 17438 - protein, 9 aa, synthetic construct
GGHGNDTLY

SEQ ID NO: 17439 - protein, 9 aa, synthetic construct
GGAGMDTLL

SEQ ID NO: 17440 - protein, 9 aa, synthetic construct
GGQGNDWVL

SEQ ID NO: 17441 - protein, 9 aa, synthetic construct
GGNGKDMMY

SEQ ID NO: 17442 - protein, 9 aa, synthetic construct
GGVGDDSLR

SEQ ID NO: 17443 - protein, 9 aa, synthetic construct
GGDGLDTLV

SEQ ID NO: 17444 - protein, 9 aa, synthetic construct
GGVGADRIE

SEQ ID NO: 17445 - protein, 9 aa, synthetic construct
GGAGSDKLD

SEQ ID NO: 17446 - protein, 9 aa, synthetic construct
GGQGNDVLH

SEQ ID NO: 17447 - protein, 9 aa, synthetic construct
GGKGGDTLI

SEQ ID NO: 17448 - protein, 9 aa, synthetic construct
GGHGSDMLI

SEQ ID NO: 17449 - protein, 9 aa, synthetic construct
GGSGNDIFQ

SEQ ID NO: 17450 - protein, 9 aa, synthetic construct
GGQGNDVIY

SEQ ID NO: 17451 - protein, 9 aa, synthetic construct
GGHGSDNLD

SEQ ID NO: 17452 - protein, 9 aa, synthetic construct
GGVGADRMR

SEQ ID NO: 17453 - protein, 9 aa, synthetic construct
GGVGADRML

SEQ ID NO: 17454 - protein, 9 aa, synthetic construct
GGKGGDTLR

SEQ ID NO: 17455 - protein, 9 aa, synthetic construct
GGEGADQVW

SEQ ID NO: 17456 - protein, 9 aa, synthetic construct
GGLGDDTYT

SEQ ID NO: 17457 - protein, 9 aa, synthetic construct
GGLGRDKLS

SEQ ID NO: 17458 - protein, 9 aa, synthetic construct
GGQGNDVLM

SEQ ID NO: 17459 - protein, 9 aa, synthetic construct
GGNGDDLII

SEQ ID NO: 17460 - protein, 9 aa, synthetic construct
GGVGDDSLE

SEQ ID NO: 17461 - protein, 9 aa, synthetic construct
GGVGADRLV

SEQ ID NO: 17462 - protein, 9 aa, synthetic construct
GGQGNDVLR

SEQ ID NO: 17463 - protein, 9 aa, synthetic construct
GGGGNDTFF

SEQ ID NO: 17464 - protein, 9 aa, synthetic construct
GGLGDDHLI

SEQ ID NO: 17465 - protein, 9 aa, synthetic construct
GGDGTDMLF

SEQ ID NO: 17466 - protein, 9 aa, synthetic construct
GGVGGDVLS

SEQ ID NO: 17467 - protein, 9 aa, synthetic construct
GGKGFDTVS

SEQ ID NO: 17468 - protein, 9 aa, synthetic construct
GGAGEDEMY

SEQ ID NO: 17469 - protein, 9 aa, synthetic construct
GGRGGDRLD

SEQ ID NO: 17470 - protein, 9 aa, synthetic construct
GGTGRDLLE

SEQ ID NO: 17471 - protein, 9 aa, synthetic construct
GGLGSDTAI

SEQ ID NO: 17472 - protein, 9 aa, synthetic construct
GGVGGDYFR

SEQ ID NO: 17473 - protein, 9 aa, synthetic construct
GGGGADVVL

SEQ ID NO: 17474 - protein, 9 aa, synthetic construct
GGAGDDIVL

SEQ ID NO: 17475 - protein, 9 aa, synthetic construct
GGAGRDIIF

SEQ ID NO: 17476 - protein, 9 aa, synthetic construct
GGRGGDRMR

SEQ ID NO: 17477 - protein, 9 aa, synthetic construct
GGVGHDALF

SEQ ID NO: 17478 - protein, 9 aa, synthetic construct
GGDGNDEIL

SEQ ID NO: 17479 - protein, 9 aa, synthetic construct
GGAGEDFLS

SEQ ID NO: 17480 - protein, 9 aa, synthetic construct
GGEGTDAVL

SEQ ID NO: 17481 - protein, 9 aa, synthetic construct
GGIGDDIID

SEQ ID NO: 17482 - protein, 9 aa, synthetic construct
GGTGRDKLF

SEQ ID NO: 17483 - protein, 9 aa, synthetic construct
GGAGRDIAL

SEQ ID NO: 17484 - protein, 9 aa, synthetic construct
GGTGRDLLG

SEQ ID NO: 17485 - protein, 9 aa, synthetic construct
GGTGRDLLI

SEQ ID NO: 17486 - protein, 9 aa, synthetic construct
GGFGDDTIF

SEQ ID NO: 17487 - protein, 9 aa, synthetic construct
GGIGDDHLE

SEQ ID NO: 17488 - protein, 9 aa, synthetic construct
GGRGFDTLS

SEQ ID NO: 17489 - protein, 9 aa, synthetic construct
GGVGGDTLT

SEQ ID NO: 17490 - protein, 9 aa, synthetic construct
GGGGADLFR

SEQ ID NO: 17491 - protein, 9 aa, synthetic construct
GGLGADTMQ

SEQ ID NO: 17492 - protein, 9 aa, synthetic construct
GGEGDDELF

SEQ ID NO: 17493 - protein, 9 aa, synthetic construct
GGVGGDTMF

SEQ ID NO: 17494 - protein, 9 aa, synthetic construct
GGIGDDFLS

SEQ ID NO: 17495 - protein, 9 aa, synthetic construct
GGDGQDNLS

SEQ ID NO: 17496 - protein, 9 aa, synthetic construct
GGVGGDVFV

SEQ ID NO: 17497 - protein, 9 aa, synthetic construct
GGNGHDTIY

SEQ ID NO: 17498 - protein, 9 aa, synthetic construct
GGAGDDIVR

SEQ ID NO: 17499 - protein, 9 aa, synthetic construct
GGTGRDLLS

SEQ ID NO: 17500 - protein, 9 aa, synthetic construct
GGKGFDVLR

SEQ ID NO: 17501 - protein, 9 aa, synthetic construct
GGEGSDYLT

SEQ ID NO: 17502 - protein, 9 aa, synthetic construct
GGRGGDLLK

SEQ ID NO: 17503 - protein, 9 aa, synthetic construct
GGFGNDTVH

SEQ ID NO: 17504 - protein, 9 aa, synthetic construct
GGEGGDYLI

SEQ ID NO: 17505 - protein, 9 aa, synthetic construct
GGRGGDTLT

SEQ ID NO: 17506 - protein, 9 aa, synthetic construct
GGEGTDFVS

SEQ ID NO: 17507 - protein, 9 aa, synthetic construct
GGTGRDILT

SEQ ID NO: 17508 - protein, 9 aa, synthetic construct
GGNGHDTFK

SEQ ID NO: 17509 - protein, 9 aa, synthetic construct
GGTGADFLY

SEQ ID NO: 17510 - protein, 9 aa, synthetic construct
GGFGDDSLV

SEQ ID NO: 17511 - protein, 9 aa, synthetic construct
GGAGEDILS

SEQ ID NO: 17512 - protein, 9 aa, synthetic construct
GGAGEDILV

SEQ ID NO: 17513 - protein, 9 aa, synthetic construct
GGAGRDGLF

SEQ ID NO: 17514 - protein, 9 aa, synthetic construct
GGAGEDILY

SEQ ID NO: 17515 - protein, 9 aa, synthetic construct
GGAGEDIMF

SEQ ID NO: 17516 - protein, 9 aa, synthetic construct
GGGGADKLN

SEQ ID NO: 17517 - protein, 9 aa, synthetic construct
GGGGNDIYL

SEQ ID NO: 17518 - protein, 9 aa, synthetic construct
GGDGSDRIS

SEQ ID NO: 17519 - protein, 9 aa, synthetic construct
GGRGHDSLY

SEQ ID NO: 17520 - protein, 9 aa, synthetic construct
GGDGTDSLD

SEQ ID NO: 17521 - protein, 9 aa, synthetic construct
GGDGSDRIQ

SEQ ID NO: 17522 - protein, 9 aa, synthetic construct
GGLGADTFI

SEQ ID NO: 17523 - protein, 9 aa, synthetic construct
GGAGDDIVD

SEQ ID NO: 17524 - protein, 9 aa, synthetic construct
GGLGADTFH

SEQ ID NO: 17525 - protein, 9 aa, synthetic construct
GGLGRDRVS

SEQ ID NO: 17526 - protein, 9 aa, synthetic construct
GGLGADTFY

SEQ ID NO: 17527 - protein, 9 aa, synthetic construct
GGEGHDALS

SEQ ID NO: 17528 - protein, 9 aa, synthetic construct
GGAGNDEAH

SEQ ID NO: 17529 - protein, 9 aa, synthetic construct
GGGGRDNLY

SEQ ID NO: 17530 - protein, 9 aa, synthetic construct
GGKGIDTLT

SEQ ID NO: 17531 - protein, 9 aa, synthetic construct
GGTGRDILN

SEQ ID NO: 17532 - protein, 9 aa, synthetic construct
GGNGLDMLD

SEQ ID NO: 17533 - protein, 9 aa, synthetic construct
GGAGEDHVH

SEQ ID NO: 17534 - protein, 9 aa, synthetic construct
GGAGEDIAD

SEQ ID NO: 17535 - protein, 9 aa, synthetic construct
GGIGDDILK

SEQ ID NO: 17536 - protein, 9 aa, synthetic construct
GGAGEDIID

SEQ ID NO: 17537 - protein, 9 aa, synthetic construct
GGAGDDIVG

SEQ ID NO: 17538 - protein, 9 aa, synthetic construct
GGTGRDGFV

SEQ ID NO: 17539 - protein, 9 aa, synthetic construct
GGLGADTIR

SEQ ID NO: 17540 - protein, 9 aa, synthetic construct
GGTGRDHLR

SEQ ID NO: 17541 - protein, 9 aa, synthetic construct
GGRGHDFLS

SEQ ID NO: 17542 - protein, 9 aa, synthetic construct
GGAGRDHLK

SEQ ID NO: 17543 - protein, 9 aa, synthetic construct
GGLGADTIQ

SEQ ID NO: 17544 - protein, 9 aa, synthetic construct
GGIGDDILR

SEQ ID NO: 17545 - protein, 9 aa, synthetic construct
GGEGNDSLH

SEQ ID NO: 17546 - protein, 9 aa, synthetic construct
GGFGNDRLV

SEQ ID NO: 17547 - protein, 9 aa, synthetic construct
GGVGGDTLN

SEQ ID NO: 17548 - protein, 9 aa, synthetic construct
GGDGSDRLT

SEQ ID NO: 17549 - protein, 9 aa, synthetic construct
GGEGNDSVG

SEQ ID NO: 17550 - protein, 9 aa, synthetic construct
GGNGDDVFY

SEQ ID NO: 17551 - protein, 9 aa, synthetic construct
GGTGRDSLV

SEQ ID NO: 17552 - protein, 9 aa, synthetic construct
GGTGRDSLS

SEQ ID NO: 17553 - protein, 9 aa, synthetic construct
GGDGQDNLQ

SEQ ID NO: 17554 - protein, 9 aa, synthetic construct
GGTGADEMY

SEQ ID NO: 17555 - protein, 9 aa, synthetic construct
GGTGRDSLE

SEQ ID NO: 17556 - protein, 9 aa, synthetic construct
GGAGRDLAS

SEQ ID NO: 17557 - protein, 9 aa, synthetic construct
GGLGDDYLF

SEQ ID NO: 17558 - protein, 9 aa, synthetic construct
GGSGLDTIL

SEQ ID NO: 17559 - protein, 9 aa, synthetic construct
GGGGADLLN

SEQ ID NO: 17560 - protein, 9 aa, synthetic construct
GGGGQDVLD

SEQ ID NO: 17561 - protein, 9 aa, synthetic construct
GGRGEDILI

SEQ ID NO: 17562 - protein, 9 aa, synthetic construct
GGAGNDDLV

SEQ ID NO: 17563 - protein, 9 aa, synthetic construct
GGRGEDILV

SEQ ID NO: 17564 - protein, 9 aa, synthetic construct
GGNGHDTLK

SEQ ID NO: 17565 - protein, 9 aa, synthetic construct
GGTGRDRLY

SEQ ID NO: 17566 - protein, 9 aa, synthetic construct
GGDGDDTIQ

SEQ ID NO: 17567 - protein, 9 aa, synthetic construct
GGHGNDKIY

SEQ ID NO: 17568 - protein, 9 aa, synthetic construct
GGLGRDRLS

SEQ ID NO: 17569 - protein, 9 aa, synthetic construct
GGEGDDALT

SEQ ID NO: 17570 - protein, 9 aa, synthetic construct
GGFGDDTID

SEQ ID NO: 17571 - protein, 9 aa, synthetic construct
GGLGADVLK

SEQ ID NO: 17572 - protein, 9 aa, synthetic construct
GGNGDDVFH

SEQ ID NO: 17573 - protein, 9 aa, synthetic construct
GGSGTDWLD

SEQ ID NO: 17574 - protein, 9 aa, synthetic construct
GGAGNDDLL

SEQ ID NO: 17575 - protein, 9 aa, synthetic construct
GGAGDDYMF

SEQ ID NO: 17576 - protein, 9 aa, synthetic construct
GGTGRDTIV

SEQ ID NO: 17577 - protein, 9 aa, synthetic construct
GGGGADLMT

SEQ ID NO: 17578 - protein, 9 aa, synthetic construct
GGEGNDSYI

SEQ ID NO: 17579 - protein, 9 aa, synthetic construct
GGLGADVLA

SEQ ID NO: 17580 - protein, 9 aa, synthetic construct
GGAGDDYVF

SEQ ID NO: 17581 - protein, 9 aa, synthetic construct
GGDGTDRLL

SEQ ID NO: 17582 - protein, 9 aa, synthetic construct
GGAGDDTYQ

SEQ ID NO: 17583 - protein, 9 aa, synthetic construct
GGRGDDVYV

SEQ ID NO: 17584 - protein, 9 aa, synthetic construct
GGLGADVLF

SEQ ID NO: 17585 - protein, 9 aa, synthetic construct
GGIGDDALI

SEQ ID NO: 17586 - protein, 9 aa, synthetic construct
GGIGTDTLE

SEQ ID NO: 17587 - protein, 9 aa, synthetic construct
GGAGDDIYH

SEQ ID NO: 17588 - protein, 9 aa, synthetic construct
GGFGDDTFV

SEQ ID NO: 17589 - protein, 9 aa, synthetic construct
GGLGADTMV

SEQ ID NO: 17590 - protein, 9 aa, synthetic construct
GGQGFDTLR

SEQ ID NO: 17591 - protein, 9 aa, synthetic construct
GGRGEDVMR

SEQ ID NO: 17592 - protein, 9 aa, synthetic construct
GGQGFDQLF

SEQ ID NO: 17593 - protein, 9 aa, synthetic construct
GGRGEDYIL

SEQ ID NO: 17594 - protein, 9 aa, synthetic construct
GGQGFDMLT

SEQ ID NO: 17595 - protein, 9 aa, synthetic construct
GGEGDDALI

SEQ ID NO: 17596 - protein, 9 aa, synthetic construct
GGLGADTVR

SEQ ID NO: 17597 - protein, 9 aa, synthetic construct
GGLGADTVQ

SEQ ID NO: 17598 - protein, 9 aa, synthetic construct
GGTGADFFV

SEQ ID NO: 17599 - protein, 9 aa, synthetic construct
GGAGSDTMA

SEQ ID NO: 17600 - protein, 9 aa, synthetic construct
GGAGSDTMD

SEQ ID NO: 17601 - protein, 9 aa, synthetic construct
GGIGDDFIF

SEQ ID NO: 17602 - protein, 9 aa, synthetic construct
GGGGNDQLW

SEQ ID NO: 17603 - protein, 9 aa, synthetic construct
GGAGEDEIK

SEQ ID NO: 17604 - protein, 9 aa, synthetic construct
GGAGRDIMV

SEQ ID NO: 17605 - protein, 9 aa, synthetic construct
GGEGNDFLE

SEQ ID NO: 17606 - protein, 9 aa, synthetic construct
GGNGADHMV

SEQ ID NO: 17607 - protein, 9 aa, synthetic construct
GGSGLDRLY

SEQ ID NO: 17608 - protein, 9 aa, synthetic construct
GGNGHDTLD

SEQ ID NO: 17609 - protein, 9 aa, synthetic construct
GGNGHDTLE

SEQ ID NO: 17610 - protein, 9 aa, synthetic construct
GGAGDDIVY

SEQ ID NO: 17611 - protein, 9 aa, synthetic construct
GGLGDDYLN

SEQ ID NO: 17612 - protein, 9 aa, synthetic construct
GGRGEDRIY

SEQ ID NO: 17613 - protein, 9 aa, synthetic construct
GGAGDDIYG

SEQ ID NO: 17614 - protein, 9 aa, synthetic construct
GGAGRDKLT

SEQ ID NO: 17615 - protein, 9 aa, synthetic construct
GGTGRDRLD

SEQ ID NO: 17616 - protein, 9 aa, synthetic construct
GGAGRDKLR

SEQ ID NO: 17617 - protein, 9 aa, synthetic construct
GGEGSDWLY

SEQ ID NO: 17618 - protein, 9 aa, synthetic construct
GGGGQDVIT

SEQ ID NO: 17619 - protein, 9 aa, synthetic construct
GGDGNDSMN

SEQ ID NO: 17620 - protein, 9 aa, synthetic construct
GGTGRDQLD

SEQ ID NO: 17621 - protein, 9 aa, synthetic construct
GGEGNDSVD

SEQ ID NO: 17622 - protein, 9 aa, synthetic construct
GGAGEDDIT

SEQ ID NO: 17623 - protein, 9 aa, synthetic construct
GGSGLDTAI

SEQ ID NO: 17624 - protein, 9 aa, synthetic construct
GGAGDDIYD

SEQ ID NO: 17625 - protein, 9 aa, synthetic construct
GGGGADLLH

SEQ ID NO: 17626 - protein, 9 aa, synthetic construct
GGGGADLLF

SEQ ID NO: 17627 - protein, 9 aa, synthetic construct
GGSGLDSLW

SEQ ID NO: 17628 - protein, 9 aa, synthetic construct
GGDGDDTFY

SEQ ID NO: 17629 - protein, 9 aa, synthetic construct
GGAGRDFLY

SEQ ID NO: 17630 - protein, 9 aa, synthetic construct
GGGGFDLLT

SEQ ID NO: 17631 - protein, 9 aa, synthetic construct
GGTGQDNMT

SEQ ID NO: 17632 - protein, 9 aa, synthetic construct
GGAGSDVFD

SEQ ID NO: 17633 - protein, 9 aa, synthetic construct
GGGGADWLV

SEQ ID NO: 17634 - protein, 9 aa, synthetic construct
GGAGQDYID

SEQ ID NO: 17635 - protein, 9 aa, synthetic construct
GGRGMDTLI

SEQ ID NO: 17636 - protein, 9 aa, synthetic construct
GGDGDDNLI

SEQ ID NO: 17637 - protein, 9 aa, synthetic construct
GGAGEDQIY

SEQ ID NO: 17638 - protein, 9 aa, synthetic construct
GGGGADWME

SEQ ID NO: 17639 - protein, 9 aa, synthetic construct
GGRGMDTYY

SEQ ID NO: 17640 - protein, 9 aa, synthetic construct
GGNGHDQLT

SEQ ID NO: 17641 - protein, 9 aa, synthetic construct
GGAGQDWLT

SEQ ID NO: 17642 - protein, 9 aa, synthetic construct
GGEGHDILL

SEQ ID NO: 17643 - protein, 9 aa, synthetic construct
GGNGHDQLL

SEQ ID NO: 17644 - protein, 9 aa, synthetic construct
GGAGQDVMT

SEQ ID NO: 17645 - protein, 9 aa, synthetic construct
GGNGHDQLF

SEQ ID NO: 17646 - protein, 9 aa, synthetic construct
GGLGSDTAS

SEQ ID NO: 17647 - protein, 9 aa, synthetic construct
GGRGNDALS

SEQ ID NO: 17648 - protein, 9 aa, synthetic construct
GGAGQDVLY

SEQ ID NO: 17649 - protein, 9 aa, synthetic construct
GGLGADRIS

SEQ ID NO: 17650 - protein, 9 aa, synthetic construct
GGNGLDRLF

SEQ ID NO: 17651 - protein, 9 aa, synthetic construct
GGFGDDSLE

SEQ ID NO: 17652 - protein, 9 aa, synthetic construct
GGTGQDSLT

SEQ ID NO: 17653 - protein, 9 aa, synthetic construct
GGAGRDALD

SEQ ID NO: 17654 - protein, 9 aa, synthetic construct
GGTGADIFQ

SEQ ID NO: 17655 - protein, 9 aa, synthetic construct
GGRGLDLLH

SEQ ID NO: 17656 - protein, 9 aa, synthetic construct
GGSGKDWLS

SEQ ID NO: 17657 - protein, 9 aa, synthetic construct
GGAGEDNLF

SEQ ID NO: 17658 - protein, 9 aa, synthetic construct
GGGGNDDLE

SEQ ID NO: 17659 - protein, 9 aa, synthetic construct
GGGGADILA

SEQ ID NO: 17660 - protein, 9 aa, synthetic construct
GGTGADIID

SEQ ID NO: 17661 - protein, 9 aa, synthetic construct
GGIGDDQID

SEQ ID NO: 17662 - protein, 9 aa, synthetic construct
GGDGDDFLM

SEQ ID NO: 17663 - protein, 9 aa, synthetic construct
GGDGNDEVD

SEQ ID NO: 17664 - protein, 9 aa, synthetic construct
GGGGNDDLD

SEQ ID NO: 17665 - protein, 9 aa, synthetic construct
GGIGDDNLS

SEQ ID NO: 17666 - protein, 9 aa, synthetic construct
GGTGQDRLT

SEQ ID NO: 17667 - protein, 9 aa, synthetic construct
GGEGADSIA

SEQ ID NO: 17668 - protein, 9 aa, synthetic construct
GGAGQDYLH

SEQ ID NO: 17669 - protein, 9 aa, synthetic construct
GGAGSDVFK

SEQ ID NO: 17670 - protein, 9 aa, synthetic construct
GGTGQDNMF

SEQ ID NO: 17671 - protein, 9 aa, synthetic construct
GGAGRDALF

SEQ ID NO: 17672 - protein, 9 aa, synthetic construct
GGEGADSIQ

SEQ ID NO: 17673 - protein, 9 aa, synthetic construct
GGRGNDELR

SEQ ID NO: 17674 - protein, 9 aa, synthetic construct
GGAGQDVID

SEQ ID NO: 17675 - protein, 9 aa, synthetic construct
GGQGDDVVS

SEQ ID NO: 17676 - protein, 9 aa, synthetic construct
GGTGQDILR

SEQ ID NO: 17677 - protein, 9 aa, synthetic construct
GGQGDDVVR

SEQ ID NO: 17678 - protein, 9 aa, synthetic construct
GGRGNDEVL

SEQ ID NO: 17679 - protein, 9 aa, synthetic construct
GGAGEDRIV

SEQ ID NO: 17680 - protein, 9 aa, synthetic construct
GGRGNDFIS

SEQ ID NO: 17681 - protein, 9 aa, synthetic construct
GGTGADILF

SEQ ID NO: 17682 - protein, 9 aa, synthetic construct
GGRGNDFLF

SEQ ID NO: 17683 - protein, 9 aa, synthetic construct
GGLGRDSVT

SEQ ID NO: 17684 - protein, 9 aa, synthetic construct
GGTGQDIIF

SEQ ID NO: 17685 - protein, 9 aa, synthetic construct
GGRGNDFLS

SEQ ID NO: 17686 - protein, 9 aa, synthetic construct
GGRGNDFVF

SEQ ID NO: 17687 - protein, 9 aa, synthetic construct
GGAGEDRLI

SEQ ID NO: 17688 - protein, 9 aa, synthetic construct
GGAGEDRLL

SEQ ID NO: 17689 - protein, 9 aa, synthetic construct
GGLGADQLN

SEQ ID NO: 17690 - protein, 9 aa, synthetic construct
GGIGDDRLN

SEQ ID NO: 17691 - protein, 9 aa, synthetic construct
GGAGDDIIE

SEQ ID NO: 17692 - protein, 9 aa, synthetic construct
GGGGGDSLV

SEQ ID NO: 17693 - protein, 9 aa, synthetic construct
GGDGDDFLT

SEQ ID NO: 17694 - protein, 9 aa, synthetic construct
GGNGADKLT

SEQ ID NO: 17695 - protein, 9 aa, synthetic construct
GGAGQDVLN

SEQ ID NO: 17696 - protein, 9 aa, synthetic construct
GGRGNDDIN

SEQ ID NO: 17697 - protein, 9 aa, synthetic construct
GGFGDDSIV

SEQ ID NO: 17698 - protein, 9 aa, synthetic construct
GGNGADLFI

SEQ ID NO: 17699 - protein, 9 aa, synthetic construct
GGEGADSIV

SEQ ID NO: 17700 - protein, 9 aa, synthetic construct
GGEGTDQIW

SEQ ID NO: 17701 - protein, 9 aa, synthetic construct
GGNGADLFR

SEQ ID NO: 17702 - protein, 9 aa, synthetic construct
GGRGNDELH

SEQ ID NO: 17703 - protein, 9 aa, synthetic construct
GGRGNDDYI

SEQ ID NO: 17704 - protein, 9 aa, synthetic construct
GGGGNDDLA

SEQ ID NO: 17705 - protein, 9 aa, synthetic construct
GGNGADLIE

SEQ ID NO: 17706 - protein, 9 aa, synthetic construct
GGAGEDRIF

SEQ ID NO: 17707 - protein, 9 aa, synthetic construct
GGEGADNIN

SEQ ID NO: 17708 - protein, 9 aa, synthetic construct
GGTGQDKIY

SEQ ID NO: 17709 - protein, 9 aa, synthetic construct
GGNGHDLVA

SEQ ID NO: 17710 - protein, 9 aa, synthetic construct
GGFGNDRLE

SEQ ID NO: 17711 - protein, 9 aa, synthetic construct
GGTGQDSLY

SEQ ID NO: 17712 - protein, 9 aa, synthetic construct
GGGGADKLI

SEQ ID NO: 17713 - protein, 9 aa, synthetic construct
GGSGLDELI

SEQ ID NO: 17714 - protein, 9 aa, synthetic construct
GGSGNDMLA

SEQ ID NO: 17715 - protein, 9 aa, synthetic construct
GGNGDDVIN

SEQ ID NO: 17716 - protein, 9 aa, synthetic construct
GGGGADKFV

SEQ ID NO: 17717 - protein, 9 aa, synthetic construct
GGTGQDYLD

SEQ ID NO: 17718 - protein, 9 aa, synthetic construct
GGNGADILV

SEQ ID NO: 17719 - protein, 9 aa, synthetic construct
GGIGDDKLI

SEQ ID NO: 17720 - protein, 9 aa, synthetic construct
GGGGADWLD

SEQ ID NO: 17721 - protein, 9 aa, synthetic construct
GGDGSDRAS

SEQ ID NO: 17722 - protein, 9 aa, synthetic construct
GGDGTDSLL

SEQ ID NO: 17723 - protein, 9 aa, synthetic construct
GGRGKDDLT

SEQ ID NO: 17724 - protein, 9 aa, synthetic construct
GGAGSDTYQ

SEQ ID NO: 17725 - protein, 9 aa, synthetic construct
GGGGQDTLI

SEQ ID NO: 17726 - protein, 9 aa, synthetic construct
GGGGADIYI

SEQ ID NO: 17727 - protein, 9 aa, synthetic construct
GGAGIDLLF

SEQ ID NO: 17728 - protein, 9 aa, synthetic construct
GGEGNDTVF

SEQ ID NO: 17729 - protein, 9 aa, synthetic construct
GGLGADSIT

SEQ ID NO: 17730 - protein, 9 aa, synthetic construct
GGTGQDVLD

SEQ ID NO: 17731 - protein, 9 aa, synthetic construct
GGAGRDELL

SEQ ID NO: 17732 - protein, 9 aa, synthetic construct
GGLGADSMF

SEQ ID NO: 17733 - protein, 9 aa, synthetic construct
GGLGADSMI

SEQ ID NO: 17734 - protein, 9 aa, synthetic construct
GGLGADSVV

SEQ ID NO: 17735 - protein, 9 aa, synthetic construct
GGRGHDVLD

SEQ ID NO: 17736 - protein, 9 aa, synthetic construct
GGRGHDVLN

SEQ ID NO: 17737 - protein, 9 aa, synthetic construct
GGEGDDALE

SEQ ID NO: 17738 - protein, 9 aa, synthetic construct
GGAGRDFLL

SEQ ID NO: 17739 - protein, 9 aa, synthetic construct
GGEGNDSLA

SEQ ID NO: 17740 - protein, 9 aa, synthetic construct
GGAGRDFIE

SEQ ID NO: 17741 - protein, 9 aa, synthetic construct
GGTGADHFV

SEQ ID NO: 17742 - protein, 9 aa, synthetic construct
GGIGTDRLY

SEQ ID NO: 17743 - protein, 9 aa, synthetic construct
GGTGRDAFR

SEQ ID NO: 17744 - protein, 9 aa, synthetic construct
GGDGNDELL

SEQ ID NO: 17745 - protein, 9 aa, synthetic construct
GGAGRDELT

SEQ ID NO: 17746 - protein, 9 aa, synthetic construct
GGAGIDLLQ

SEQ ID NO: 17747 - protein, 9 aa, synthetic construct
GGAGRDELR

SEQ ID NO: 17748 - protein, 9 aa, synthetic construct
GGAGSDTYA

SEQ ID NO: 17749 - protein, 9 aa, synthetic construct
GGEGDDLLM

SEQ ID NO: 17750 - protein, 9 aa, synthetic construct
GGLGADSMN

SEQ ID NO: 17751 - protein, 9 aa, synthetic construct
GGAGEDLLY

SEQ ID NO: 17752 - protein, 9 aa, synthetic construct
GGDGQDRIF

SEQ ID NO: 17753 - protein, 9 aa, synthetic construct
GGLGADRLS

SEQ ID NO: 17754 - protein, 9 aa, synthetic construct
GGRGKDLID

SEQ ID NO: 17755 - protein, 9 aa, synthetic construct
GGNGADKFV

SEQ ID NO: 17756 - protein, 9 aa, synthetic construct
GGQGDDYLD

SEQ ID NO: 17757 - protein, 9 aa, synthetic construct
GGTGQDTLH

SEQ ID NO: 17758 - protein, 9 aa, synthetic construct
GGLGADRMS

SEQ ID NO: 17759 - protein, 9 aa, synthetic construct
GGLGADRML

SEQ ID NO: 17760 - protein, 9 aa, synthetic construct
GGRGKDTYD

SEQ ID NO: 17761 - protein, 9 aa, synthetic construct
GGFGDDSLL

SEQ ID NO: 17762 - protein, 9 aa, synthetic construct
GGDGTDSLS

SEQ ID NO: 17763 - protein, 9 aa, synthetic construct
GGFGDDSLI

SEQ ID NO: 17764 - protein, 9 aa, synthetic construct
GGSGKDYIE

SEQ ID NO: 17765 - protein, 9 aa, synthetic construct
GGVGHDTLN

SEQ ID NO: 17766 - protein, 9 aa, synthetic construct
GGTGQDTIT

SEQ ID NO: 17767 - protein, 9 aa, synthetic construct
GGTGQDTFI

SEQ ID NO: 17768 - protein, 9 aa, synthetic construct
GGGGADILK

SEQ ID NO: 17769 - protein, 9 aa, synthetic construct
GGEGTDKVA

SEQ ID NO: 17770 - protein, 9 aa, synthetic construct
GGQGDDYIE

SEQ ID NO: 17771 - protein, 9 aa, synthetic construct
GGDGSDNYN

SEQ ID NO: 17772 - protein, 9 aa, synthetic construct
GGSGNDMLG

SEQ ID NO: 17773 - protein, 9 aa, synthetic construct
GGAGNDELA

SEQ ID NO: 17774 - protein, 9 aa, synthetic construct
GGRGKDRVK

SEQ ID NO: 17775 - protein, 9 aa, synthetic construct
GGGGQDTIY

SEQ ID NO: 17776 - protein, 9 aa, synthetic construct
GGDGDDFLE

SEQ ID NO: 17777 - protein, 9 aa, synthetic construct
GGAGSDTYS

SEQ ID NO: 17778 - protein, 9 aa, synthetic construct
GGAGRDDLR

SEQ ID NO: 17779 - protein, 9 aa, synthetic construct
GGAGNDEIW

SEQ ID NO: 17780 - protein, 9 aa, synthetic construct
GGEGDDELN

SEQ ID NO: 17781 - protein, 9 aa, synthetic construct
GGEGHDIAH

SEQ ID NO: 17782 - protein, 9 aa, synthetic construct
GGDGSDQLR

SEQ ID NO: 17783 - protein, 9 aa, synthetic construct
GGDGDDFLH

SEQ ID NO: 17784 - protein, 9 aa, synthetic construct
GGLGTDTAE

SEQ ID NO: 17785 - protein, 9 aa, synthetic construct
GGDGSDQLI

SEQ ID NO: 17786 - protein, 9 aa, synthetic construct
GGLGEDKLY

SEQ ID NO: 17787 - protein, 9 aa, synthetic construct
GGVGHDNLF

SEQ ID NO: 17788 - protein, 9 aa, synthetic construct
GGTGQDTLY

SEQ ID NO: 17789 - protein, 9 aa, synthetic construct
GGTGQDTLV

SEQ ID NO: 17790 - protein, 9 aa, synthetic construct
GGSGTDVFV

SEQ ID NO: 17791 - protein, 9 aa, synthetic construct
GGGGNDDLG

SEQ ID NO: 17792 - protein, 9 aa, synthetic construct
GGRGDDVLL

SEQ ID NO: 17793 - protein, 9 aa, synthetic construct
GGRGDDVYR

SEQ ID NO: 17794 - protein, 9 aa, synthetic construct
GGDGSDSVF

SEQ ID NO: 17795 - protein, 9 aa, synthetic construct
GGTGSDRFI

SEQ ID NO: 17796 - protein, 9 aa, synthetic construct
GGDGLDLLD

SEQ ID NO: 17797 - protein, 9 aa, synthetic construct
GGLGDDEIK

SEQ ID NO: 17798 - protein, 9 aa, synthetic construct
GGAGDDKLR

SEQ ID NO: 17799 - protein, 9 aa, synthetic construct
GGAGRDRMI

SEQ ID NO: 17800 - protein, 9 aa, synthetic construct
GGAGRDRMF

SEQ ID NO: 17801 - protein, 9 aa, synthetic construct
GGTGSDSML

SEQ ID NO: 17802 - protein, 9 aa, synthetic construct
GGTGSDSLS

SEQ ID NO: 17803 - protein, 9 aa, synthetic construct
GGDGNDALQ

SEQ ID NO: 17804 - protein, 9 aa, synthetic construct
GGTGSDSLF

SEQ ID NO: 17805 - protein, 9 aa, synthetic construct
GGNGDDILL

SEQ ID NO: 17806 - protein, 9 aa, synthetic construct
GGDGSDTLE

SEQ ID NO: 17807 - protein, 9 aa, synthetic construct
GGSGNDAIN

SEQ ID NO: 17808 - protein, 9 aa, synthetic construct
GGDGNDALV

SEQ ID NO: 17809 - protein, 9 aa, synthetic construct
GGTGSDRME

SEQ ID NO: 17810 - protein, 9 aa, synthetic construct
GGRGDDHLL

SEQ ID NO: 17811 - protein, 9 aa, synthetic construct
GGEGDDLMI

SEQ ID NO: 17812 - protein, 9 aa, synthetic construct
GGGGNDQVY

SEQ ID NO: 17813 - protein, 9 aa, synthetic construct
GGDGDDEMY

SEQ ID NO: 17814 - protein, 9 aa, synthetic construct
GGLGDDELA

SEQ ID NO: 17815 - protein, 9 aa, synthetic construct
GGAGSDTAL

SEQ ID NO: 17816 - protein, 9 aa, synthetic construct
GGTGSDTAI

SEQ ID NO: 17817 - protein, 9 aa, synthetic construct
GGVGEDQLW

SEQ ID NO: 17818 - protein, 9 aa, synthetic construct
GGAGRDSIF

SEQ ID NO: 17819 - protein, 9 aa, synthetic construct
GGAGRDSIE

SEQ ID NO: 17820 - protein, 9 aa, synthetic construct
GGGGNDELH

SEQ ID NO: 17821 - protein, 9 aa, synthetic construct
GGIGADSLD

SEQ ID NO: 17822 - protein, 9 aa, synthetic construct
GGRGDDELN

SEQ ID NO: 17823 - protein, 9 aa, synthetic construct
GGTGSDTAL

SEQ ID NO: 17824 - protein, 9 aa, synthetic construct
GGGGFDQMT

SEQ ID NO: 17825 - protein, 9 aa, synthetic construct
GGGGFDTID

SEQ ID NO: 17826 - protein, 9 aa, synthetic construct
GGEGNDFIS

SEQ ID NO: 17827 - protein, 9 aa, synthetic construct
GGDGFDTYN

SEQ ID NO: 17828 - protein, 9 aa, synthetic construct
GGEGGDIIV

SEQ ID NO: 17829 - protein, 9 aa, synthetic construct
GGTGADALT

SEQ ID NO: 17830 - protein, 9 aa, synthetic construct
GGDGDDDAA

SEQ ID NO: 17831 - protein, 9 aa, synthetic construct
GGTGSDSMS

SEQ ID NO: 17832 - protein, 9 aa, synthetic construct
GGEGKDTFT

SEQ ID NO: 17833 - protein, 9 aa, synthetic construct
GGAGRDRLQ

SEQ ID NO: 17834 - protein, 9 aa, synthetic construct
GGTGSDRAS

SEQ ID NO: 17835 - protein, 9 aa, synthetic construct
GGAGDDVVT

SEQ ID NO: 17836 - protein, 9 aa, synthetic construct
GGAGDDVMF

SEQ ID NO: 17837 - protein, 9 aa, synthetic construct
GGAGRDRIS

SEQ ID NO: 17838 - protein, 9 aa, synthetic construct
GGIGVDIFD

SEQ ID NO: 17839 - protein, 9 aa, synthetic construct
GGVGEDSLV

SEQ ID NO: 17840 - protein, 9 aa, synthetic construct
GGRGDDKLK

SEQ ID NO: 17841 - protein, 9 aa, synthetic construct
GGRGDDKLS

SEQ ID NO: 17842 - protein, 9 aa, synthetic construct
GGDGSDSVH

SEQ ID NO: 17843 - protein, 9 aa, synthetic construct
GGAGIDWVS

SEQ ID NO: 17844 - protein, 9 aa, synthetic construct
GGRGDDKMK

SEQ ID NO: 17845 - protein, 9 aa, synthetic construct
GGGGADNLD

SEQ ID NO: 17846 - protein, 9 aa, synthetic construct
GGDGNDAVN

SEQ ID NO: 17847 - protein, 9 aa, synthetic construct
GGDGNDAVR

SEQ ID NO: 17848 - protein, 9 aa, synthetic construct
GGAGIDWVV

SEQ ID NO: 17849 - protein, 9 aa, synthetic construct
GGLGDDAYV

SEQ ID NO: 17850 - protein, 9 aa, synthetic construct
GGAGDDVVE

SEQ ID NO: 17851 - protein, 9 aa, synthetic construct
GGIGADTFK

SEQ ID NO: 17852 - protein, 9 aa, synthetic construct
GGIGADTFR

SEQ ID NO: 17853 - protein, 9 aa, synthetic construct
GGFGNDTLH

SEQ ID NO: 17854 - protein, 9 aa, synthetic construct
GGGGADNLH

SEQ ID NO: 17855 - protein, 9 aa, synthetic construct
GGGGNDIIV

SEQ ID NO: 17856 - protein, 9 aa, synthetic construct
GGRGDDIYV

SEQ ID NO: 17857 - protein, 9 aa, synthetic construct
GGEGDDVFQ

SEQ ID NO: 17858 - protein, 9 aa, synthetic construct
GGGGFDTIY

SEQ ID NO: 17859 - protein, 9 aa, synthetic construct
GGRGDDIIF

SEQ ID NO: 17860 - protein, 9 aa, synthetic construct
GGTGSDQLY

SEQ ID NO: 17861 - protein, 9 aa, synthetic construct
GGRGDDILA

SEQ ID NO: 17862 - protein, 9 aa, synthetic construct
GGLGDDDLK

SEQ ID NO: 17863 - protein, 9 aa, synthetic construct
GGAGNDAYI

SEQ ID NO: 17864 - protein, 9 aa, synthetic construct
GGTGSDQFV

SEQ ID NO: 17865 - protein, 9 aa, synthetic construct
GGRGDDILS

SEQ ID NO: 17866 - protein, 9 aa, synthetic construct
GGNGHDWLY

SEQ ID NO: 17867 - protein, 9 aa, synthetic construct
GGNGKDWLY

SEQ ID NO: 17868 - protein, 9 aa, synthetic construct
GGSGNDLVD

SEQ ID NO: 17869 - protein, 9 aa, synthetic construct
GGGGNDIIS

SEQ ID NO: 17870 - protein, 9 aa, synthetic construct
GGAGDDVMY

SEQ ID NO: 17871 - protein, 9 aa, synthetic construct
GGFGNDTLE

SEQ ID NO: 17872 - protein, 9 aa, synthetic construct
GGFGNDTLF

SEQ ID NO: 17873 - protein, 9 aa, synthetic construct
GGAGRDRIY

SEQ ID NO: 17874 - protein, 9 aa, synthetic construct
GGIGADSIT

SEQ ID NO: 17875 - protein, 9 aa, synthetic construct
GGKGHDTLE

SEQ ID NO: 17876 - protein, 9 aa, synthetic construct
GGAGRDSIV

SEQ ID NO: 17877 - protein, 9 aa, synthetic construct
GGTGADALI

SEQ ID NO: 17878 - protein, 9 aa, synthetic construct
GGIGADRMY

SEQ ID NO: 17879 - protein, 9 aa, synthetic construct
GGTGSDVMT

SEQ ID NO: 17880 - protein, 9 aa, synthetic construct
GGGGNDIIE

SEQ ID NO: 17881 - protein, 9 aa, synthetic construct
GGSGYDVYW

SEQ ID NO: 17882 - protein, 9 aa, synthetic construct
GGGGADQLN

SEQ ID NO: 17883 - protein, 9 aa, synthetic construct
GGGGNDELL

SEQ ID NO: 17884 - protein, 9 aa, synthetic construct
GGAGNDALW

SEQ ID NO: 17885 - protein, 9 aa, synthetic construct
GGAGRDTFL

SEQ ID NO: 17886 - protein, 9 aa, synthetic construct
GGAGDDKMV

SEQ ID NO: 17887 - protein, 9 aa, synthetic construct
GGTGSDVLN

SEQ ID NO: 17888 - protein, 9 aa, synthetic construct
GGLGRDQLR

SEQ ID NO: 17889 - protein, 9 aa, synthetic construct
GGDGFDTLL

SEQ ID NO: 17890 - protein, 9 aa, synthetic construct
GGLGDDFVA

SEQ ID NO: 17891 - protein, 9 aa, synthetic construct
GGRGADVLA

SEQ ID NO: 17892 - protein, 9 aa, synthetic construct
GGRGADVLD

SEQ ID NO: 17893 - protein, 9 aa, synthetic construct
GGRGADVLK

SEQ ID NO: 17894 - protein, 9 aa, synthetic construct
GGRGADVLS

SEQ ID NO: 17895 - protein, 9 aa, synthetic construct
GGDGGDTLA

SEQ ID NO: 17896 - protein, 9 aa, synthetic construct
GGAGIDRLH

SEQ ID NO: 17897 - protein, 9 aa, synthetic construct
GGEGSDTYQ

SEQ ID NO: 17898 - protein, 9 aa, synthetic construct
GGDGDDVLW

SEQ ID NO: 17899 - protein, 9 aa, synthetic construct
GGIGADRLT

SEQ ID NO: 17900 - protein, 9 aa, synthetic construct
GGDGDDELL

SEQ ID NO: 17901 - protein, 9 aa, synthetic construct
GGNGIDNLF

SEQ ID NO: 17902 - protein, 9 aa, synthetic construct
GGGGNDTFH

SEQ ID NO: 17903 - protein, 9 aa, synthetic construct
GGLGDDGLY

SEQ ID NO: 17904 - protein, 9 aa, synthetic construct
GGRGADTIS

SEQ ID NO: 17905 - protein, 9 aa, synthetic construct
GGAGDDTYS

SEQ ID NO: 17906 - protein, 9 aa, synthetic construct
GGSGNDDIQ

SEQ ID NO: 17907 - protein, 9 aa, synthetic construct
GGEGSDNLA

SEQ ID NO: 17908 - protein, 9 aa, synthetic construct
GGIGADRLV

SEQ ID NO: 17909 - protein, 9 aa, synthetic construct
GGAGDDVAF

SEQ ID NO: 17910 - protein, 9 aa, synthetic construct
GGEGDDEIS

SEQ ID NO: 17911 - protein, 9 aa, synthetic construct
GGTGSDWLD

SEQ ID NO: 17912 - protein, 9 aa, synthetic construct
GGAGIDRLI

SEQ ID NO: 17913 - protein, 9 aa, synthetic construct
GGGGNDELR

SEQ ID NO: 17914 - protein, 9 aa, synthetic construct
GGGGHDRMG

SEQ ID NO: 17915 - protein, 9 aa, synthetic construct
GGAGDDVFY

SEQ ID NO: 17916 - protein, 9 aa, synthetic construct
GGKGHDTID

SEQ ID NO: 17917 - protein, 9 aa, synthetic construct
GGRGADVMT

SEQ ID NO: 17918 - protein, 9 aa, synthetic construct
GGDGNDAIY

SEQ ID NO: 17919 - protein, 9 aa, synthetic construct
GGTGSDTIV

SEQ ID NO: 17920 - protein, 9 aa, synthetic construct
GGTGSDTIS

SEQ ID NO: 17921 - protein, 9 aa, synthetic construct
GGQGHDQLF

SEQ ID NO: 17922 - protein, 9 aa, synthetic construct
GGAGNDAVF

SEQ ID NO: 17923 - protein, 9 aa, synthetic construct
GGLGDDFIN

SEQ ID NO: 17924 - protein, 9 aa, synthetic construct
GGRGDDALV

SEQ ID NO: 17925 - protein, 9 aa, synthetic construct
GGDGDDDIA

SEQ ID NO: 17926 - protein, 9 aa, synthetic construct
GGAGRDSLL

SEQ ID NO: 17927 - protein, 9 aa, synthetic construct
GGAGIDRFL

SEQ ID NO: 17928 - protein, 9 aa, synthetic construct
GGQGHDLLY

SEQ ID NO: 17929 - protein, 9 aa, synthetic construct
GGGGADQAD

SEQ ID NO: 17930 - protein, 9 aa, synthetic construct
GGTGADALD

SEQ ID NO: 17931 - protein, 9 aa, synthetic construct
GGAGDDVIW

SEQ ID NO: 17932 - protein, 9 aa, synthetic construct
GGTGSDTII

SEQ ID NO: 17933 - protein, 9 aa, synthetic construct
GGRGDDDIN

SEQ ID NO: 17934 - protein, 9 aa, synthetic construct
GGTGADALF

SEQ ID NO: 17935 - protein, 9 aa, synthetic construct
GGRGDDALG

SEQ ID NO: 17936 - protein, 9 aa, synthetic construct
GGRGDDAIW

SEQ ID NO: 17937 - protein, 9 aa, synthetic construct
GGLGDDVYM

SEQ ID NO: 17938 - protein, 9 aa, synthetic construct
GGFGDDTLT

SEQ ID NO: 17939 - protein, 9 aa, synthetic construct
GGGGADQIY

SEQ ID NO: 17940 - protein, 9 aa, synthetic construct
GGTGSDTYH

SEQ ID NO: 17941 - protein, 9 aa, synthetic construct
GGTGSDTVT

SEQ ID NO: 17942 - protein, 9 aa, synthetic construct
GGTGSDTVL

SEQ ID NO: 17943 - protein, 9 aa, synthetic construct
GGGGADQID

SEQ ID NO: 17944 - protein, 9 aa, synthetic construct
GGRGADYIE

SEQ ID NO: 17945 - protein, 9 aa, synthetic construct
GGGGRDLLS

SEQ ID NO: 17946 - protein, 9 aa, synthetic construct
GGFGDDYME

SEQ ID NO: 17947 - protein, 9 aa, synthetic construct
GGAGRDSLW

SEQ ID NO: 17948 - protein, 9 aa, synthetic construct
GGEGNDTML

SEQ ID NO: 17949 - protein, 9 aa, synthetic construct
GGTGSDTMV

SEQ ID NO: 17950 - protein, 9 aa, synthetic construct
GGAGIDRFV

SEQ ID NO: 17951 - protein, 9 aa, synthetic construct
GGEGADVLF

SEQ ID NO: 17952 - protein, 9 aa, synthetic construct
GGDGDDTME

SEQ ID NO: 17953 - protein, 9 aa, synthetic construct
GGRGCDTLV

SEQ ID NO: 17954 - protein, 9 aa, synthetic construct
GGSGNDLMM

SEQ ID NO: 17955 - protein, 9 aa, synthetic construct
GGTGSDLVV

SEQ ID NO: 17956 - protein, 9 aa, synthetic construct
GGRGDDKLV

SEQ ID NO: 17957 - protein, 9 aa, synthetic construct
GGNGHDWLN

SEQ ID NO: 17958 - protein, 9 aa, synthetic construct
GGVGFDLLI

SEQ ID NO: 17959 - protein, 9 aa, synthetic construct
GGRGDDSLE

SEQ ID NO: 17960 - protein, 9 aa, synthetic construct
GGIGADTMR

SEQ ID NO: 17961 - protein, 9 aa, synthetic construct
GGIGADTMS

SEQ ID NO: 17962 - protein, 9 aa, synthetic construct
GGAGIDNLY

SEQ ID NO: 17963 - protein, 9 aa, synthetic construct
GGEGSDVLF

SEQ ID NO: 17964 - protein, 9 aa, synthetic construct
GGIGADTVI

SEQ ID NO: 17965 - protein, 9 aa, synthetic construct
GGQGGDMID

SEQ ID NO: 17966 - protein, 9 aa, synthetic construct
GGDGNDSVL

SEQ ID NO: 17967 - protein, 9 aa, synthetic construct
GGNGADEFF

SEQ ID NO: 17968 - protein, 9 aa, synthetic construct
GGDGDDFIL

SEQ ID NO: 17969 - protein, 9 aa, synthetic construct
GGGGFDNIY

SEQ ID NO: 17970 - protein, 9 aa, synthetic construct
GGGGQDYIE

SEQ ID NO: 17971 - protein, 9 aa, synthetic construct
GGIGADVFI

SEQ ID NO: 17972 - protein, 9 aa, synthetic construct
GGRGDDSYI

SEQ ID NO: 17973 - protein, 9 aa, synthetic construct
GGDGDDLFY

SEQ ID NO: 17974 - protein, 9 aa, synthetic construct
GGMGNDTVS

SEQ ID NO: 17975 - protein, 9 aa, synthetic construct
GGIGADVFV

SEQ ID NO: 17976 - protein, 9 aa, synthetic construct
GGQGGDRIV

SEQ ID NO: 17977 - protein, 9 aa, synthetic construct
GGIGADTMM

SEQ ID NO: 17978 - protein, 9 aa, synthetic construct
GGAGNDDIE

SEQ ID NO: 17979 - protein, 9 aa, synthetic construct
GGSGMDVAD

SEQ ID NO: 17980 - protein, 9 aa, synthetic construct
GGSGNDLVN

SEQ ID NO: 17981 - protein, 9 aa, synthetic construct
GGGGNDTFY

SEQ ID NO: 17982 - protein, 9 aa, synthetic construct
GGTGSDHIS

SEQ ID NO: 17983 - protein, 9 aa, synthetic construct
GGAGRDNIA

SEQ ID NO: 17984 - protein, 9 aa, synthetic construct
GGDGNDDLI

SEQ ID NO: 17985 - protein, 9 aa, synthetic construct
GGKGHDTYV

SEQ ID NO: 17986 - protein, 9 aa, synthetic construct
GGNGADDLN

SEQ ID NO: 17987 - protein, 9 aa, synthetic construct
GGTGADDLS

SEQ ID NO: 17988 - protein, 9 aa, synthetic construct
GGAGDDWLW

SEQ ID NO: 17989 - protein, 9 aa, synthetic construct
GGAGDDWLQ

SEQ ID NO: 17990 - protein, 9 aa, synthetic construct
GGNGKDYLY

SEQ ID NO: 17991 - protein, 9 aa, synthetic construct
GGDGNDSVN

SEQ ID NO: 17992 - protein, 9 aa, synthetic construct
GGAGDDWLR

SEQ ID NO: 17993 - protein, 9 aa, synthetic construct
GGAGRDMLN

SEQ ID NO: 17994 - protein, 9 aa, synthetic construct
GGRGDDRVY

SEQ ID NO: 17995 - protein, 9 aa, synthetic construct
GGGGNDSLE

SEQ ID NO: 17996 - protein, 9 aa, synthetic construct
GGDGSDTFA

SEQ ID NO: 17997 - protein, 9 aa, synthetic construct
GGEGSDLLY

SEQ ID NO: 17998 - protein, 9 aa, synthetic construct
GGAGNDDIM

SEQ ID NO: 17999 - protein, 9 aa, synthetic construct
GGHGNDLIY

SEQ ID NO: 18000 - protein, 9 aa, synthetic construct
GGTGRDVLT

SEQ ID NO: 18001 - protein, 9 aa, synthetic construct
GGTGRDVLN

SEQ ID NO: 18002 - protein, 9 aa, synthetic construct
GGDGSDSYT

SEQ ID NO: 18003 - protein, 9 aa, synthetic construct
GGRGDDVIA

SEQ ID NO: 18004 - protein, 9 aa, synthetic construct
GGDGGDTLF

SEQ ID NO: 18005 - protein, 9 aa, synthetic construct
GGLGDDYLA

SEQ ID NO: 18006 - protein, 9 aa, synthetic construct
GGTGRDVLI

SEQ ID NO: 18007 - protein, 9 aa, synthetic construct
GGTGRDVLH

SEQ ID NO: 18008 - protein, 9 aa, synthetic construct
GGTGRDVLW

SEQ ID NO: 18009 - protein, 9 aa, synthetic construct
GGTGADEIH

SEQ ID NO: 18010 - protein, 9 aa, synthetic construct
GGHGNDLIE

SEQ ID NO: 18011 - protein, 9 aa, synthetic construct
GGRGDDVIS

SEQ ID NO: 18012 - protein, 9 aa, synthetic construct
GGTGRDVLE

SEQ ID NO: 18013 - protein, 9 aa, synthetic construct
GGAGDDYLK

SEQ ID NO: 18014 - protein, 9 aa, synthetic construct
GGNGADEMY

SEQ ID NO: 18015 - protein, 9 aa, synthetic construct
GGAGDDKAS

SEQ ID NO: 18016 - protein, 9 aa, synthetic construct
GGTGRDVLV

SEQ ID NO: 18017 - protein, 9 aa, synthetic construct
GGRGDDTVS

SEQ ID NO: 18018 - protein, 9 aa, synthetic construct
GGLGADVMQ

SEQ ID NO: 18019 - protein, 9 aa, synthetic construct
GGRGDDTLK

SEQ ID NO: 18020 - protein, 9 aa, synthetic construct
GGFGDDTII

SEQ ID NO: 18021 - protein, 9 aa, synthetic construct
GGRGDDTIN

SEQ ID NO: 18022 - protein, 9 aa, synthetic construct
GGEGSDVMI

SEQ ID NO: 18023 - protein, 9 aa, synthetic construct
GGHGNDLLE

SEQ ID NO: 18024 - protein, 9 aa, synthetic construct
GGAGRDLVD

SEQ ID NO: 18025 - protein, 9 aa, synthetic construct
GGIGADVLD

SEQ ID NO: 18026 - protein, 9 aa, synthetic construct
GGTGRDYLT

SEQ ID NO: 18027 - protein, 9 aa, synthetic construct
GGAGDDYII

SEQ ID NO: 18028 - protein, 9 aa, synthetic construct
GGAGDDYIV

SEQ ID NO: 18029 - protein, 9 aa, synthetic construct
GGKGHDVLS

SEQ ID NO: 18030 - protein, 9 aa, synthetic construct
GGKGHDVVD

SEQ ID NO: 18031 - protein, 9 aa, synthetic construct
GGNGHDTLT

SEQ ID NO: 18032 - protein, 9 aa, synthetic construct
GGRGDDTMS

SEQ ID NO: 18033 - protein, 9 aa, synthetic construct
GGGGADLMW

SEQ ID NO: 18034 - protein, 9 aa, synthetic construct
GGLGTDTID

SEQ ID NO: 18035 - protein, 9 aa, synthetic construct
GGAGDDYIT

SEQ ID NO: 18036 - protein, 9 aa, synthetic construct
GGRGDDRLF

SEQ ID NO: 18037 - protein, 9 aa, synthetic construct
GGVGDDQIL

SEQ ID NO: 18038 - protein, 9 aa, synthetic construct
GGQGGDVLY

SEQ ID NO: 18039 - protein, 9 aa, synthetic construct
GGSGNDLVL

SEQ ID NO: 18040 - protein, 9 aa, synthetic construct
GGTGSDLLG

SEQ ID NO: 18041 - protein, 9 aa, synthetic construct
GGVGEDYLA

SEQ ID NO: 18042 - protein, 9 aa, synthetic construct
GGTGSDLLD

SEQ ID NO: 18043 - protein, 9 aa, synthetic construct
GGAGRDNLY

SEQ ID NO: 18044 - protein, 9 aa, synthetic construct
GGLGADYLS

SEQ ID NO: 18045 - protein, 9 aa, synthetic construct
GGAGRDNYY

SEQ ID NO: 18046 - protein, 9 aa, synthetic construct
GGDGNDDIG

SEQ ID NO: 18047 - protein, 9 aa, synthetic construct
GGDGSDTIE

SEQ ID NO: 18048 - protein, 9 aa, synthetic construct
GGRGDDLVL

SEQ ID NO: 18049 - protein, 9 aa, synthetic construct
GGDGSDTII

SEQ ID NO: 18050 - protein, 9 aa, synthetic construct
GGFGDDTLA

SEQ ID NO: 18051 - protein, 9 aa, synthetic construct
GGAGRDQMH

SEQ ID NO: 18052 - protein, 9 aa, synthetic construct
GGNGADALV

SEQ ID NO: 18053 - protein, 9 aa, synthetic construct
GGRGDDQLY

SEQ ID NO: 18054 - protein, 9 aa, synthetic construct
GGRGDDQID

SEQ ID NO: 18055 - protein, 9 aa, synthetic construct
GGAGRDQFV

SEQ ID NO: 18056 - protein, 9 aa, synthetic construct
GGGGNDEIW

SEQ ID NO: 18057 - protein, 9 aa, synthetic construct
GGGGFDTLL

SEQ ID NO: 18058 - protein, 9 aa, synthetic construct
GGDGQDLLV

SEQ ID NO: 18059 - protein, 9 aa, synthetic construct
GGAGRDQIH

SEQ ID NO: 18060 - protein, 9 aa, synthetic construct
GGAGDDKLH

SEQ ID NO: 18061 - protein, 9 aa, synthetic construct
GGSGMDTLT

SEQ ID NO: 18062 - protein, 9 aa, synthetic construct
GGRGDDNLD

SEQ ID NO: 18063 - protein, 9 aa, synthetic construct
GGRGDDLYQ

SEQ ID NO: 18064 - protein, 9 aa, synthetic construct
GGTGSDILI

SEQ ID NO: 18065 - protein, 9 aa, synthetic construct
GGEGDDVFL

SEQ ID NO: 18066 - protein, 9 aa, synthetic construct
GGTGADDFI

SEQ ID NO: 18067 - protein, 9 aa, synthetic construct
GGFGDDTIY

SEQ ID NO: 18068 - protein, 9 aa, synthetic construct
GGDGNDDLH

SEQ ID NO: 18069 - protein, 9 aa, synthetic construct
GGAGRDQLQ

SEQ ID NO: 18070 - protein, 9 aa, synthetic construct
GGDGNDDLG

SEQ ID NO: 18071 - protein, 9 aa, synthetic construct
GGSGMDRLE

SEQ ID NO: 18072 - protein, 9 aa, synthetic construct
GGFGDDTLI

SEQ ID NO: 18073 - protein, 9 aa, synthetic construct
GGDGTDRAS

SEQ ID NO: 18074 - protein, 9 aa, synthetic construct
GGLGDDAIR

SEQ ID NO: 18075 - protein, 9 aa, synthetic construct
GGEGNDTMT

SEQ ID NO: 18076 - protein, 9 aa, synthetic construct
GGEGSDVID

SEQ ID NO: 18077 - protein, 9 aa, synthetic construct
GGNGADALL

SEQ ID NO: 18078 - protein, 9 aa, synthetic construct
GGAGSDTIG

SEQ ID NO: 18079 - protein, 9 aa, synthetic construct
GGTGSDLLQ

SEQ ID NO: 18080 - protein, 9 aa, synthetic construct
GGEGGDIIA

SEQ ID NO: 18081 - protein, 9 aa, synthetic construct
GGAGRDQLH

SEQ ID NO: 18082 - protein, 9 aa, synthetic construct
GGIGADTIF

SEQ ID NO: 18083 - protein, 9 aa, synthetic construct
GGAGRDRFA

SEQ ID NO: 18084 - protein, 9 aa, synthetic construct
GGAGRDNLG

SEQ ID NO: 18085 - protein, 9 aa, synthetic construct
GGVGEDTLF

SEQ ID NO: 18086 - protein, 9 aa, synthetic construct
GGTGSDIID

SEQ ID NO: 18087 - protein, 9 aa, synthetic construct
GGNGDDILH

SEQ ID NO: 18088 - protein, 9 aa, synthetic construct
GGDGLDILV

SEQ ID NO: 18089 - protein, 9 aa, synthetic construct
GGSGMDTMH

SEQ ID NO: 18090 - protein, 9 aa, synthetic construct
GGAGMDQLS

SEQ ID NO: 18091 - protein, 9 aa, synthetic construct
GGDGGDDLN

SEQ ID NO: 18092 - protein, 9 aa, synthetic construct
GGMGADRLF

SEQ ID NO: 18093 - protein, 9 aa, synthetic construct
GGGGIDAMI

SEQ ID NO: 18094 - protein, 9 aa, synthetic construct
GGDGGDTIV

SEQ ID NO: 18095 - protein, 9 aa, synthetic construct
GGGGHDRID

SEQ ID NO: 18096 - protein, 9 aa, synthetic construct
GGLGRDELR

SEQ ID NO: 18097 - protein, 9 aa, synthetic construct
GGLGSDIFR

SEQ ID NO: 18098 - protein, 9 aa, synthetic construct
GGLGSDRMS

SEQ ID NO: 18099 - protein, 9 aa, synthetic construct
GGDGGDILN

SEQ ID NO: 18100 - protein, 9 aa, synthetic construct
GGEGDDQVS

SEQ ID NO: 18101 - protein, 9 aa, synthetic construct
GGLGSDSID

SEQ ID NO: 18102 - protein, 9 aa, synthetic construct
GGLGSDRMI

SEQ ID NO: 18103 - protein, 9 aa, synthetic construct
GGLGSDTYK

SEQ ID NO: 18104 - protein, 9 aa, synthetic construct
GGDGGDILQ

SEQ ID NO: 18105 - protein, 9 aa, synthetic construct
GGLGSDIFI

SEQ ID NO: 18106 - protein, 9 aa, synthetic construct
GGGGHDVLS

SEQ ID NO: 18107 - protein, 9 aa, synthetic construct
GGDGGDTLW

SEQ ID NO: 18108 - protein, 9 aa, synthetic construct
GGDGGDHMN

SEQ ID NO: 18109 - protein, 9 aa, synthetic construct
GGDGGDTLQ

SEQ ID NO: 18110 - protein, 9 aa, synthetic construct
GGLGQDYLV

SEQ ID NO: 18111 - protein, 9 aa, synthetic construct
GGEGDDLFN

SEQ ID NO: 18112 - protein, 9 aa, synthetic construct
GGLGSDTVD

SEQ ID NO: 18113 - protein, 9 aa, synthetic construct
GGLGRDILN

SEQ ID NO: 18114 - protein, 9 aa, synthetic construct
GGLGVDLLT

SEQ ID NO: 18115 - protein, 9 aa, synthetic construct
GGLGSDILQ

SEQ ID NO: 18116 - protein, 9 aa, synthetic construct
GGLGSDIFA

SEQ ID NO: 18117 - protein, 9 aa, synthetic construct
GGDGGDTLH

SEQ ID NO: 18118 - protein, 9 aa, synthetic construct
GGLGVDLLQ

SEQ ID NO: 18119 - protein, 9 aa, synthetic construct
GGDGGDIIS

SEQ ID NO: 18120 - protein, 9 aa, synthetic construct
GGDGGDTLI

SEQ ID NO: 18121 - protein, 9 aa, synthetic construct
GGLGSDTVS

SEQ ID NO: 18122 - protein, 9 aa, synthetic construct
GGDGFDFAS

SEQ ID NO: 18123 - protein, 9 aa, synthetic construct
GGGGIDALS

SEQ ID NO: 18124 - protein, 9 aa, synthetic construct
GGDGFDTII

SEQ ID NO: 18125 - protein, 9 aa, synthetic construct
GGDGGDILD

SEQ ID NO: 18126 - protein, 9 aa, synthetic construct
GGLGVDQLS

SEQ ID NO: 18127 - protein, 9 aa, synthetic construct
GGDGGDTIR

SEQ ID NO: 18128 - protein, 9 aa, synthetic construct
GGLGSDSIG

SEQ ID NO: 18129 - protein, 9 aa, synthetic construct
GGLGNDYMK

SEQ ID NO: 18130 - protein, 9 aa, synthetic construct
GGMGADRLA

SEQ ID NO: 18131 - protein, 9 aa, synthetic construct
GGLGVDMLT

SEQ ID NO: 18132 - protein, 9 aa, synthetic construct
GGLGSDILR

SEQ ID NO: 18133 - protein, 9 aa, synthetic construct
GGLGSDTLW

SEQ ID NO: 18134 - protein, 9 aa, synthetic construct
GGMGADRLM

SEQ ID NO: 18135 - protein, 9 aa, synthetic construct
GGLGSDTYI

SEQ ID NO: 18136 - protein, 9 aa, synthetic construct
GGLGSDTVI

SEQ ID NO: 18137 - protein, 9 aa, synthetic construct
GGLGSDIVL

SEQ ID NO: 18138 - protein, 9 aa, synthetic construct
GGDGGDTVT

SEQ ID NO: 18139 - protein, 9 aa, synthetic construct
GGDGGDTIT

SEQ ID NO: 18140 - protein, 9 aa, synthetic construct
GGLGRDALT

SEQ ID NO: 18141 - protein, 9 aa, synthetic construct
GGGGHDQIF

SEQ ID NO: 18142 - protein, 9 aa, synthetic construct
GGEGDDNLS

SEQ ID NO: 18143 - protein, 9 aa, synthetic construct
GGLGRDHLA

SEQ ID NO: 18144 - protein, 9 aa, synthetic construct
GGLGSDMLS

SEQ ID NO: 18145 - protein, 9 aa, synthetic construct
GGLGRDFYS

SEQ ID NO: 18146 - protein, 9 aa, synthetic construct
GGLGVDHLF

SEQ ID NO: 18147 - protein, 9 aa, synthetic construct
GGEGDDNVD

SEQ ID NO: 18148 - protein, 9 aa, synthetic construct
GGLGSDRMT

SEQ ID NO: 18149 - protein, 9 aa, synthetic construct
GGLGVDILI

SEQ ID NO: 18150 - protein, 9 aa, synthetic construct
GGMGADRLI

SEQ ID NO: 18151 - protein, 9 aa, synthetic construct
GGLGRDTFF

SEQ ID NO: 18152 - protein, 9 aa, synthetic construct
GGLGVDQLT

SEQ ID NO: 18153 - protein, 9 aa, synthetic construct
GGLGYDEYH

SEQ ID NO: 18154 - protein, 9 aa, synthetic construct
GGDGFDRAT

SEQ ID NO: 18155 - protein, 9 aa, synthetic construct
GGDGEDWVR

SEQ ID NO: 18156 - protein, 9 aa, synthetic construct
GGGGIDTVR

SEQ ID NO: 18157 - protein, 9 aa, synthetic construct
GGLGTDLLT

SEQ ID NO: 18158 - protein, 9 aa, synthetic construct
GGLGQDDLV

SEQ ID NO: 18159 - protein, 9 aa, synthetic construct
GGLGTDTIY

SEQ ID NO: 18160 - protein, 9 aa, synthetic construct
GGDGGDELD

SEQ ID NO: 18161 - protein, 9 aa, synthetic construct
GGGGHDTIM

SEQ ID NO: 18162 - protein, 9 aa, synthetic construct
GGLGTDLLD

SEQ ID NO: 18163 - protein, 9 aa, synthetic construct
GGDGFDTLF

SEQ ID NO: 18164 - protein, 9 aa, synthetic construct
GGLGRDVYA

SEQ ID NO: 18165 - protein, 9 aa, synthetic construct
GGLGRDRLI

SEQ ID NO: 18166 - protein, 9 aa, synthetic construct
GGGGIDIAD

SEQ ID NO: 18167 - protein, 9 aa, synthetic construct
GGLGRDRLF

SEQ ID NO: 18168 - protein, 9 aa, synthetic construct
GGLGSDLYQ

SEQ ID NO: 18169 - protein, 9 aa, synthetic construct
GGGGIDTIY

SEQ ID NO: 18170 - protein, 9 aa, synthetic construct
GGDGFDQLY

SEQ ID NO: 18171 - protein, 9 aa, synthetic construct
GGLGRDVMR

SEQ ID NO: 18172 - protein, 9 aa, synthetic construct
GGLGQDRFY

SEQ ID NO: 18173 - protein, 9 aa, synthetic construct
GGDGGDMLK

SEQ ID NO: 18174 - protein, 9 aa, synthetic construct
GGDGHDALT

SEQ ID NO: 18175 - protein, 9 aa, synthetic construct
GGDGGDWLY

SEQ ID NO: 18176 - protein, 9 aa, synthetic construct
GGEGDDRIM

SEQ ID NO: 18177 - protein, 9 aa, synthetic construct
GGLGRDVLI

SEQ ID NO: 18178 - protein, 9 aa, synthetic construct
GGLGWDTLN

SEQ ID NO: 18179 - protein, 9 aa, synthetic construct
GGEGDDQMA

SEQ ID NO: 18180 - protein, 9 aa, synthetic construct
GGDGGDMLA

SEQ ID NO: 18181 - protein, 9 aa, synthetic construct
GGGGIDTMI

SEQ ID NO: 18182 - protein, 9 aa, synthetic construct
GGGGIDTMQ

SEQ ID NO: 18183 - protein, 9 aa, synthetic construct
GGEGDDQLH

SEQ ID NO: 18184 - protein, 9 aa, synthetic construct
GGLGSDTFF

SEQ ID NO: 18185 - protein, 9 aa, synthetic construct
GGGGHDKIN

SEQ ID NO: 18186 - protein, 9 aa, synthetic construct
GGEGDDRIT

SEQ ID NO: 18187 - protein, 9 aa, synthetic construct
GGLGSDLYY

SEQ ID NO: 18188 - protein, 9 aa, synthetic construct
GGEGDDQID

SEQ ID NO: 18189 - protein, 9 aa, synthetic construct
GGLGTDTFV

SEQ ID NO: 18190 - protein, 9 aa, synthetic construct
GGGGIDTVT

SEQ ID NO: 18191 - protein, 9 aa, synthetic construct
GGDGGDAID

SEQ ID NO: 18192 - protein, 9 aa, synthetic construct
GGDGFDLLC

SEQ ID NO: 18193 - protein, 9 aa, synthetic construct
GGEGDDLIQ

SEQ ID NO: 18194 - protein, 9 aa, synthetic construct
GGEGDDMIV

SEQ ID NO: 18195 - protein, 9 aa, synthetic construct
GGDGGDRLN

SEQ ID NO: 18196 - protein, 9 aa, synthetic construct
GGDGGDRLR

SEQ ID NO: 18197 - protein, 9 aa, synthetic construct
GGLGRDQMW

SEQ ID NO: 18198 - protein, 9 aa, synthetic construct
GGLGSDLIS

SEQ ID NO: 18199 - protein, 9 aa, synthetic construct
GGLGQDSLI

SEQ ID NO: 18200 - protein, 9 aa, synthetic construct
GGEGDDMLA

SEQ ID NO: 18201 - protein, 9 aa, synthetic construct
GGLGTDILF

SEQ ID NO: 18202 - protein, 9 aa, synthetic construct
GGEGDDMLD

SEQ ID NO: 18203 - protein, 9 aa, synthetic construct
GGDGGDFLD

SEQ ID NO: 18204 - protein, 9 aa, synthetic construct
GGGGIDLVT

SEQ ID NO: 18205 - protein, 9 aa, synthetic construct
GGLGRDQLS

SEQ ID NO: 18206 - protein, 9 aa, synthetic construct
GGLGYDLAL

SEQ ID NO: 18207 - protein, 9 aa, synthetic construct
GGLGYDIMY

SEQ ID NO: 18208 - protein, 9 aa, synthetic construct
GGLGRDRFV

SEQ ID NO: 18209 - protein, 9 aa, synthetic construct
GGLGTDIVR

SEQ ID NO: 18210 - protein, 9 aa, synthetic construct
GGGGIDIAA

SEQ ID NO: 18211 - protein, 9 aa, synthetic construct
GGLGRDYID

SEQ ID NO: 18212 - protein, 9 aa, synthetic construct
GGLGRDYLF

SEQ ID NO: 18213 - protein, 9 aa, synthetic construct
GGLGSDRLA

SEQ ID NO: 18214 - protein, 9 aa, synthetic construct
GGLGTDKLG

SEQ ID NO: 18215 - protein, 9 aa, synthetic construct
GGLGSDPAL

SEQ ID NO: 18216 - protein, 9 aa, synthetic construct
GGLGQDRLY

SEQ ID NO: 18217 - protein, 9 aa, synthetic construct
GGLGYDILT

SEQ ID NO: 18218 - protein, 9 aa, synthetic construct
GGLGYDIAL

SEQ ID NO: 18219 - protein, 9 aa, synthetic construct
GGGGIDTIT

SEQ ID NO: 18220 - protein, 9 aa, synthetic construct
GGDGEDVFT

SEQ ID NO: 18221 - protein, 9 aa, synthetic construct
GGLGRDRLA

SEQ ID NO: 18222 - protein, 9 aa, synthetic construct
GGDGFDTLH

SEQ ID NO: 18223 - protein, 9 aa, synthetic construct
GGDGGDWLA

SEQ ID NO: 18224 - protein, 9 aa, synthetic construct
GGDGGDMML

SEQ ID NO: 18225 - protein, 9 aa, synthetic construct
GGDGGDELF

SEQ ID NO: 18226 - protein, 9 aa, synthetic construct
GGLGSDAID

SEQ ID NO: 18227 - protein, 9 aa, synthetic construct
GGLGQDMLV

SEQ ID NO: 18228 - protein, 9 aa, synthetic construct
GGDGFDFAD

SEQ ID NO: 18229 - protein, 9 aa, synthetic construct
GGLGVDTME

SEQ ID NO: 18230 - protein, 9 aa, synthetic construct
GGDGFDMVM

SEQ ID NO: 18231 - protein, 9 aa, synthetic construct
GGLGRDSLS

SEQ ID NO: 18232 - protein, 9 aa, synthetic construct
GGLGRDTLH

SEQ ID NO: 18233 - protein, 9 aa, synthetic construct
GGLGRDTLL

SEQ ID NO: 18234 - protein, 9 aa, synthetic construct
GGEGDDLVF

SEQ ID NO: 18235 - protein, 9 aa, synthetic construct
GGDGGDRFV

SEQ ID NO: 18236 - protein, 9 aa, synthetic construct
GGDGGDYLY

SEQ ID NO: 18237 - protein, 9 aa, synthetic construct
GGGGHDVLE

SEQ ID NO: 18238 - protein, 9 aa, synthetic construct
GGDGGDRIY

SEQ ID NO: 18239 - protein, 9 aa, synthetic construct
GGLGQDLLV

SEQ ID NO: 18240 - protein, 9 aa, synthetic construct
GGLGTDTAI

SEQ ID NO: 18241 - protein, 9 aa, synthetic construct
GGLGTDTAR

SEQ ID NO: 18242 - protein, 9 aa, synthetic construct
GGEGDDQLL

SEQ ID NO: 18243 - protein, 9 aa, synthetic construct
GGLGVDTMI

SEQ ID NO: 18244 - protein, 9 aa, synthetic construct
GGDGGDYMF

SEQ ID NO: 18245 - protein, 9 aa, synthetic construct
GGGGHDLLN

SEQ ID NO: 18246 - protein, 9 aa, synthetic construct
GGLGQDILS

SEQ ID NO: 18247 - protein, 9 aa, synthetic construct
GGGGHDLLV

SEQ ID NO: 18248 - protein, 9 aa, synthetic construct
GGLGRDTFD

SEQ ID NO: 18249 - protein, 9 aa, synthetic construct
GGDGFDYAS

SEQ ID NO: 18250 - protein, 9 aa, synthetic construct
GGGGHDSID

SEQ ID NO: 18251 - protein, 9 aa, synthetic construct
GGDGFDLVS

SEQ ID NO: 18252 - protein, 9 aa, synthetic construct
GGLGRDSLV

SEQ ID NO: 18253 - protein, 9 aa, synthetic construct
GGLGRDTIK

SEQ ID NO: 18254 - protein, 9 aa, synthetic construct
GGLGVDTYI

SEQ ID NO: 18255 - protein, 9 aa, synthetic construct
GGLGQDKLH

SEQ ID NO: 18256 - protein, 9 aa, synthetic construct
GGEGDDLVS

SEQ ID NO: 18257 - protein, 9 aa, synthetic construct
GGGGHDSLE

SEQ ID NO: 18258 - protein, 9 aa, synthetic construct
GGGGIDIVS

SEQ ID NO: 18259 - protein, 9 aa, synthetic construct
GGDGHDAID

SEQ ID NO: 18260 - protein, 9 aa, synthetic construct
GGLGTDSVF

SEQ ID NO: 18261 - protein, 9 aa, synthetic construct
GGGGHDSLI

SEQ ID NO: 18262 - protein, 9 aa, synthetic construct
GGLGRDTLR

SEQ ID NO: 18263 - protein, 9 aa, synthetic construct
GGLGQDRFI

SEQ ID NO: 18264 - protein, 9 aa, synthetic construct
GGLGVDTLY

SEQ ID NO: 18265 - protein, 9 aa, synthetic construct
GGLGTDTFT

SEQ ID NO: 18266 - protein, 9 aa, synthetic construct
GGEGDDLYE

SEQ ID NO: 18267 - protein, 9 aa, synthetic construct
GGGGIDTMA

SEQ ID NO: 18268 - protein, 9 aa, synthetic construct
GGLGRDTMW

SEQ ID NO: 18269 - protein, 9 aa, synthetic construct
GGDGGDNVS

SEQ ID NO: 18270 - protein, 9 aa, synthetic construct
GGDGGDELL

SEQ ID NO: 18271 - protein, 9 aa, synthetic construct
GGEGDDLYI

SEQ ID NO: 18272 - protein, 9 aa, synthetic construct
GGLGSDQLW

SEQ ID NO: 18273 - protein, 9 aa, synthetic construct
GGGGIDILD

SEQ ID NO: 18274 - protein, 9 aa, synthetic construct
GGDGGDWVV

SEQ ID NO: 18275 - protein, 9 aa, synthetic construct
GGDGHDALS

SEQ ID NO: 18276 - protein, 9 aa, synthetic construct
GGEGDDNIN

SEQ ID NO: 18277 - protein, 9 aa, synthetic construct
GGDGGDNIQ

SEQ ID NO: 18278 - protein, 9 aa, synthetic construct
GGEGDDNLD

SEQ ID NO: 18279 - protein, 9 aa, synthetic construct
GGLGWDTAS

SEQ ID NO: 18280 - protein, 9 aa, synthetic construct
GGDGHDALH

SEQ ID NO: 18281 - protein, 9 aa, synthetic construct
GGDGEDVLI

SEQ ID NO: 18282 - protein, 9 aa, synthetic construct
GGLGRDTMI

SEQ ID NO: 18283 - protein, 9 aa, synthetic construct
GGLGSDLLA

SEQ ID NO: 18284 - protein, 9 aa, synthetic construct
GGDGEDVLR

SEQ ID NO: 18285 - protein, 9 aa, synthetic construct
GGDGFDQAS

SEQ ID NO: 18286 - protein, 9 aa, synthetic construct
GGLGTDQMF

SEQ ID NO: 18287 - protein, 9 aa, synthetic construct
GGLGSDQLV

SEQ ID NO: 18288 - protein, 9 aa, synthetic construct
GGLGVDYAA

SEQ ID NO: 18289 - protein, 9 aa, synthetic construct
GGGGHDVVD

SEQ ID NO: 18290 - protein, 9 aa, synthetic construct
GGDGFDYID

SEQ ID NO: 18291 - protein, 9 aa, synthetic construct
GGGGHDLLD

SEQ ID NO: 18292 - protein, 9 aa, synthetic construct
GGLGTDTAY

SEQ ID NO: 18293 - protein, 9 aa, synthetic construct
GGDGFDYLI

SEQ ID NO: 18294 - protein, 9 aa, synthetic construct
GGGGHDRVY

SEQ ID NO: 18295 - protein, 9 aa, synthetic construct
GGLGRDTMA

SEQ ID NO: 18296 - protein, 9 aa, synthetic construct
GGDGGDQFF

SEQ ID NO: 18297 - protein, 9 aa, synthetic construct
GGGGHDLLE

SEQ ID NO: 18298 - protein, 9 aa, synthetic construct
GGDGFDTLI

SEQ ID NO: 18299 - protein, 9 aa, synthetic construct
GGDGEDYLD

SEQ ID NO: 18300 - protein, 9 aa, synthetic construct
GGLGVDQMF

SEQ ID NO: 18301 - protein, 9 aa, synthetic construct
GGLGVDRLL

SEQ ID NO: 18302 - protein, 9 aa, synthetic construct
GGLGVDALY

SEQ ID NO: 18303 - protein, 9 aa, synthetic construct
GGLGSDFLK

SEQ ID NO: 18304 - protein, 9 aa, synthetic construct
GGLGVDRLN

SEQ ID NO: 18305 - protein, 9 aa, synthetic construct
GGDGFDTLY

SEQ ID NO: 18306 - protein, 9 aa, synthetic construct
GGMGADGLF

SEQ ID NO: 18307 - protein, 9 aa, synthetic construct
GGLGPDFLY

SEQ ID NO: 18308 - protein, 9 aa, synthetic construct
GGLGSDFLT

SEQ ID NO: 18309 - protein, 9 aa, synthetic construct
GGLGQDTMA

SEQ ID NO: 18310 - protein, 9 aa, synthetic construct
GGLGSDTIY

SEQ ID NO: 18311 - protein, 9 aa, synthetic construct
GGDGEDTLD

SEQ ID NO: 18312 - protein, 9 aa, synthetic construct
GGGGHDILD

SEQ ID NO: 18313 - protein, 9 aa, synthetic construct
GGMGADILH

SEQ ID NO: 18314 - protein, 9 aa, synthetic construct
GGLGSDFVN

SEQ ID NO: 18315 - protein, 9 aa, synthetic construct
GGLGRDKLR

SEQ ID NO: 18316 - protein, 9 aa, synthetic construct
GGLGNDYYV

SEQ ID NO: 18317 - protein, 9 aa, synthetic construct
GGDGGDALY

SEQ ID NO: 18318 - protein, 9 aa, synthetic construct
GGLGRDKLW

SEQ ID NO: 18319 - protein, 9 aa, synthetic construct
GGLGVDAIA

SEQ ID NO: 18320 - protein, 9 aa, synthetic construct
GGLGTDWVV

SEQ ID NO: 18321 - protein, 9 aa, synthetic construct
GGLGSDELQ

SEQ ID NO: 18322 - protein, 9 aa, synthetic construct
GGLGPDLAL

SEQ ID NO: 18323 - protein, 9 aa, synthetic construct
GGDGGDKLL

SEQ ID NO: 18324 - protein, 9 aa, synthetic construct
GGGGIDRFV

SEQ ID NO: 18325 - protein, 9 aa, synthetic construct
GGLGTDVMN

SEQ ID NO: 18326 - protein, 9 aa, synthetic construct
GGGGHDRLE

SEQ ID NO: 18327 - protein, 9 aa, synthetic construct
GGEGDDRIY

SEQ ID NO: 18328 - protein, 9 aa, synthetic construct
GGLGVDRME

SEQ ID NO: 18329 - protein, 9 aa, synthetic construct
GGGGHDRLD

SEQ ID NO: 18330 - protein, 9 aa, synthetic construct
GGLGSDTIV

SEQ ID NO: 18331 - protein, 9 aa, synthetic construct
GGDGFDIFV

SEQ ID NO: 18332 - protein, 9 aa, synthetic construct
GGGGIDRIS

SEQ ID NO: 18333 - protein, 9 aa, synthetic construct
GGGGIDVMI

SEQ ID NO: 18334 - protein, 9 aa, synthetic construct
GGGGHDMMF

SEQ ID NO: 18335 - protein, 9 aa, synthetic construct
GGDGEDTIT

SEQ ID NO: 18336 - protein, 9 aa, synthetic construct
GGDGGDEIY

SEQ ID NO: 18337 - protein, 9 aa, synthetic construct
GGDGGDSLV

SEQ ID NO: 18338 - protein, 9 aa, synthetic construct
GGEGDDQMV

SEQ ID NO: 18339 - protein, 9 aa, synthetic construct
GGMGADLLR

SEQ ID NO: 18340 - protein, 9 aa, synthetic construct
GGGGIDTAI

SEQ ID NO: 18341 - protein, 9 aa, synthetic construct
GGDGFDGLS

SEQ ID NO: 18342 - protein, 9 aa, synthetic construct
GGDGFDTVV

SEQ ID NO: 18343 - protein, 9 aa, synthetic construct
GGLGNDYVS

SEQ ID NO: 18344 - protein, 9 aa, synthetic construct
GGDGGDTIF

SEQ ID NO: 18345 - protein, 9 aa, synthetic construct
GGLGSDVFE

SEQ ID NO: 18346 - protein, 9 aa, synthetic construct
GGDGFDGIH

SEQ ID NO: 18347 - protein, 9 aa, synthetic construct
GGLGSDGFA

SEQ ID NO: 18348 - protein, 9 aa, synthetic construct
GGGGHDVFR

SEQ ID NO: 18349 - protein, 9 aa, synthetic construct
GGLGSDTYY

SEQ ID NO: 18350 - protein, 9 aa, synthetic construct
GGLGSDKII

SEQ ID NO: 18351 - protein, 9 aa, synthetic construct
GGDGGDILT

SEQ ID NO: 18352 - protein, 9 aa, synthetic construct
GGEGDDLLG

SEQ ID NO: 18353 - protein, 9 aa, synthetic construct
GGLGVDQMT

SEQ ID NO: 18354 - protein, 9 aa, synthetic construct
GGGGIDTAR

SEQ ID NO: 18355 - protein, 9 aa, synthetic construct
GGLGQDVMT

SEQ ID NO: 18356 - protein, 9 aa, synthetic construct
GGDGFDIAA

SEQ ID NO: 18357 - protein, 9 aa, synthetic construct
GGLGSDVIT

SEQ ID NO: 18358 - protein, 9 aa, synthetic construct
GGMGADIMT

SEQ ID NO: 18359 - protein, 9 aa, synthetic construct
GGDGEDTII

SEQ ID NO: 18360 - protein, 9 aa, synthetic construct
GGGGHDTYV

SEQ ID NO: 18361 - protein, 9 aa, synthetic construct
GGLGVDRLE

SEQ ID NO: 18362 - protein, 9 aa, synthetic construct
GGDGGDVIY

SEQ ID NO: 18363 - protein, 9 aa, synthetic construct
GGLGVDEMQ

SEQ ID NO: 18364 - protein, 9 aa, synthetic construct
GGGGHDIFV

SEQ ID NO: 18365 - protein, 9 aa, synthetic construct
GGLGSDTLH

SEQ ID NO: 18366 - protein, 9 aa, synthetic construct
GGLGSDRLS

SEQ ID NO: 18367 - protein, 9 aa, synthetic construct
GGMGADLLF

SEQ ID NO: 18368 - protein, 9 aa, synthetic construct
GGDGFDTFF

SEQ ID NO: 18369 - protein, 9 aa, synthetic construct
GGLGSDVII

SEQ ID NO: 18370 - protein, 9 aa, synthetic construct
GGLGQDVLK

SEQ ID NO: 18371 - protein, 9 aa, synthetic construct
GGGGHDNLY

SEQ ID NO: 18372 - protein, 9 aa, synthetic construct
GGDGGDLID

SEQ ID NO: 18373 - protein, 9 aa, synthetic construct
GGLGSDSLN

SEQ ID NO: 18374 - protein, 9 aa, synthetic construct
GGLGTDILD

SEQ ID NO: 18375 - protein, 9 aa, synthetic construct
GGDGGDVMS

SEQ ID NO: 18376 - protein, 9 aa, synthetic construct
GGEGDDLMD

SEQ ID NO: 18377 - protein, 9 aa, synthetic construct
GGLGYDRVL

SEQ ID NO: 18378 - protein, 9 aa, synthetic construct
GGLGTDTMA

SEQ ID NO: 18379 - protein, 9 aa, synthetic construct
GGDGEDTVN

SEQ ID NO: 18380 - protein, 9 aa, synthetic construct
GGLGVDTAS

SEQ ID NO: 18381 - protein, 9 aa, synthetic construct
GGDGGDAIW

SEQ ID NO: 18382 - protein, 9 aa, synthetic construct
GGLGQDTAI

SEQ ID NO: 18383 - protein, 9 aa, synthetic construct
GGGGHDYLD

SEQ ID NO: 18384 - protein, 9 aa, synthetic construct
GGLGVDTAI

SEQ ID NO: 18385 - protein, 9 aa, synthetic construct
GGDGEDTVH

SEQ ID NO: 18386 - protein, 9 aa, synthetic construct
GGLGVDTAG

SEQ ID NO: 18387 - protein, 9 aa, synthetic construct
GGDGFDSIY

SEQ ID NO: 18388 - protein, 9 aa, synthetic construct
GGLGSDKVY

SEQ ID NO: 18389 - protein, 9 aa, synthetic construct
GGDGFDSLD

SEQ ID NO: 18390 - protein, 9 aa, synthetic construct
GGDGFDSLF

SEQ ID NO: 18391 - protein, 9 aa, synthetic construct
GGDGGDSAV

SEQ ID NO: 18392 - protein, 9 aa, synthetic construct
GGEGDDQMF

SEQ ID NO: 18393 - protein, 9 aa, synthetic construct
GGLGVDTFQ

SEQ ID NO: 18394 - protein, 9 aa, synthetic construct
GGDGGDRVV

SEQ ID NO: 18395 - protein, 9 aa, synthetic construct
GGDGGDRLY

SEQ ID NO: 18396 - protein, 9 aa, synthetic construct
GGLGQDSLM

SEQ ID NO: 18397 - protein, 9 aa, synthetic construct
GGLGSDALK

SEQ ID NO: 18398 - protein, 9 aa, synthetic construct
GGDGGDLLQ

SEQ ID NO: 18399 - protein, 9 aa, synthetic construct
GGLGSDALY

SEQ ID NO: 18400 - protein, 9 aa, synthetic construct
GGGGHDVLW

SEQ ID NO: 18401 - protein, 9 aa, synthetic construct
GGGGHDMLV

SEQ ID NO: 18402 - protein, 9 aa, synthetic construct
GGDGHDEII

SEQ ID NO: 18403 - protein, 9 aa, synthetic construct
GGLGPDTLD

SEQ ID NO: 18404 - protein, 9 aa, synthetic construct
GGLGYDRLQ

SEQ ID NO: 18405 - protein, 9 aa, synthetic construct
GGLGTDTLV

SEQ ID NO: 18406 - protein, 9 aa, synthetic construct
GGDGHDEIH

SEQ ID NO: 18407 - protein, 9 aa, synthetic construct
GGDGGDDID

SEQ ID NO: 18408 - protein, 9 aa, synthetic construct
GGLGTDFLL

SEQ ID NO: 18409 - protein, 9 aa, synthetic construct
GGLGTDALF

SEQ ID NO: 18410 - protein, 9 aa, synthetic construct
GGDGFDSLH

SEQ ID NO: 18411 - protein, 9 aa, synthetic construct
GGLGSDVLQ

SEQ ID NO: 18412 - protein, 9 aa, synthetic construct
GGLGQDTFH

SEQ ID NO: 18413 - protein, 9 aa, synthetic construct
GGDGGDLIQ

SEQ ID NO: 18414 - protein, 9 aa, synthetic construct
GGLGSDRLI

SEQ ID NO: 18415 - protein, 9 aa, synthetic construct
GGDGFDTIV

SEQ ID NO: 18416 - protein, 9 aa, synthetic construct
GGLGRDLLQ

SEQ ID NO: 18417 - protein, 9 aa, synthetic construct
GGLGSDVLS

SEQ ID NO: 18418 - protein, 9 aa, synthetic construct
GGDGFDILW

SEQ ID NO: 18419 - protein, 9 aa, synthetic construct
GGDGGDVLN

SEQ ID NO: 18420 - protein, 9 aa, synthetic construct
GGDGEDTLK

SEQ ID NO: 18421 - protein, 9 aa, synthetic construct
GGLGQDTLE

SEQ ID NO: 18422 - protein, 9 aa, synthetic construct
GGLGSDDYH

SEQ ID NO: 18423 - protein, 9 aa, synthetic construct
GGDGGDSLF

SEQ ID NO: 18424 - protein, 9 aa, synthetic construct
GGGGIDRAD

SEQ ID NO: 18425 - protein, 9 aa, synthetic construct
GGGGHDRLL

SEQ ID NO: 18426 - protein, 9 aa, synthetic construct
GGLGRDLLA

SEQ ID NO: 18427 - protein, 9 aa, synthetic construct
GGDGEDYMI

SEQ ID NO: 18428 - protein, 9 aa, synthetic construct
GGDGFDTAL

SEQ ID NO: 18429 - protein, 9 aa, synthetic construct
GGLGYDYAI

SEQ ID NO: 18430 - protein, 9 aa, synthetic construct
GGLGRDLLV

SEQ ID NO: 18431 - protein, 9 aa, synthetic construct
GGDGFDTLT

SEQ ID NO: 18432 - protein, 9 aa, synthetic construct
GGDGGDVLY

SEQ ID NO: 18433 - protein, 9 aa, synthetic construct
GGLGSDSMT

SEQ ID NO: 18434 - protein, 9 aa, synthetic construct
GGLGSDKLV

SEQ ID NO: 18435 - protein, 9 aa, synthetic construct
GGGGHDVIE

SEQ ID NO: 18436 - protein, 9 aa, synthetic construct
GGLGQDTFV

SEQ ID NO: 18437 - protein, 9 aa, synthetic construct
GGGGIDQAS

SEQ ID NO: 18438 - protein, 9 aa, synthetic construct
GGLGSDWLD

SEQ ID NO: 18439 - protein, 9 aa, synthetic construct
GGLGSDTIE

SEQ ID NO: 18440 - protein, 9 aa, synthetic construct
GGDGGDSIT

SEQ ID NO: 18441 - protein, 9 aa, synthetic construct
GGLGTDTVS

SEQ ID NO: 18442 - protein, 9 aa, synthetic construct
GGLGSDDLS

SEQ ID NO: 18443 - protein, 9 aa, synthetic construct
GGDGGDVLV

SEQ ID NO: 18444 - protein, 9 aa, synthetic construct
GGDGFDIVS

SEQ ID NO: 18445 - protein, 9 aa, synthetic construct
GGDGGDVLS

SEQ ID NO: 18446 - protein, 9 aa, synthetic construct
GGLGSDWIF

SEQ ID NO: 18447 - protein, 9 aa, synthetic construct
GGPGDDTLQ

SEQ ID NO: 18448 - protein, 9 aa, synthetic construct
GGLGNDYLW

SEQ ID NO: 18449 - protein, 9 aa, synthetic construct
GGDGRDTLE

SEQ ID NO: 18450 - protein, 9 aa, synthetic construct
GGIGNDELY

SEQ ID NO: 18451 - protein, 9 aa, synthetic construct
GGIGNDELR

SEQ ID NO: 18452 - protein, 9 aa, synthetic construct
GGDGRDTLM

SEQ ID NO: 18453 - protein, 9 aa, synthetic construct
GGIGNDDLR

SEQ ID NO: 18454 - protein, 9 aa, synthetic construct
GGIGNDDLN

SEQ ID NO: 18455 - protein, 9 aa, synthetic construct
GGGGNDYIR

SEQ ID NO: 18456 - protein, 9 aa, synthetic construct
GGGGNDYIS

SEQ ID NO: 18457 - protein, 9 aa, synthetic construct
GGDGRDTMR

SEQ ID NO: 18458 - protein, 9 aa, synthetic construct
GGIGNDALL

SEQ ID NO: 18459 - protein, 9 aa, synthetic construct
GGIGMDFLN

SEQ ID NO: 18460 - protein, 9 aa, synthetic construct
GGDGRDVFG

SEQ ID NO: 18461 - protein, 9 aa, synthetic construct
GGDGRDVFV

SEQ ID NO: 18462 - protein, 9 aa, synthetic construct
GGDGRDVIF

SEQ ID NO: 18463 - protein, 9 aa, synthetic construct
GGIGLDTMN

SEQ ID NO: 18464 - protein, 9 aa, synthetic construct
GGDGRDVIL

SEQ ID NO: 18465 - protein, 9 aa, synthetic construct
GGDGRDTLG

SEQ ID NO: 18466 - protein, 9 aa, synthetic construct
GGDGRDTIV

SEQ ID NO: 18467 - protein, 9 aa, synthetic construct
GGIGNDKLA

SEQ ID NO: 18468 - protein, 9 aa, synthetic construct
GGDGRDTIS

SEQ ID NO: 18469 - protein, 9 aa, synthetic construct
GGDGRDSLW

SEQ ID NO: 18470 - protein, 9 aa, synthetic construct
GGDGRDSVL

SEQ ID NO: 18471 - protein, 9 aa, synthetic construct
GGDGRDTAS

SEQ ID NO: 18472 - protein, 9 aa, synthetic construct
GGGGNDWVW

SEQ ID NO: 18473 - protein, 9 aa, synthetic construct
GGDGRDTFA

SEQ ID NO: 18474 - protein, 9 aa, synthetic construct
GGIGNDIID

SEQ ID NO: 18475 - protein, 9 aa, synthetic construct
GGIGNDIAI

SEQ ID NO: 18476 - protein, 9 aa, synthetic construct
GGIGNDHLT

SEQ ID NO: 18477 - protein, 9 aa, synthetic construct
GGGGNDYFI

SEQ ID NO: 18478 - protein, 9 aa, synthetic construct
GGDGRDTIH

SEQ ID NO: 18479 - protein, 9 aa, synthetic construct
GGDGRDTII

SEQ ID NO: 18480 - protein, 9 aa, synthetic construct
GGIGNDGLD

SEQ ID NO: 18481 - protein, 9 aa, synthetic construct
GGIGNDFMV

SEQ ID NO: 18482 - protein, 9 aa, synthetic construct
GGIGNDFLT

SEQ ID NO: 18483 - protein, 9 aa, synthetic construct
GGDGRDTIR

SEQ ID NO: 18484 - protein, 9 aa, synthetic construct
GGGGNDYLL

SEQ ID NO: 18485 - protein, 9 aa, synthetic construct
GGIGLDTID

SEQ ID NO: 18486 - protein, 9 aa, synthetic construct
GGIGLDTFV

SEQ ID NO: 18487 - protein, 9 aa, synthetic construct
GGIGLDRIF

SEQ ID NO: 18488 - protein, 9 aa, synthetic construct
GGDGRDYID

SEQ ID NO: 18489 - protein, 9 aa, synthetic construct
GGIGIDVLN

SEQ ID NO: 18490 - protein, 9 aa, synthetic construct
GGIGIDVLA

SEQ ID NO: 18491 - protein, 9 aa, synthetic construct
GGDGRDYLL

SEQ ID NO: 18492 - protein, 9 aa, synthetic construct
GGEGADTIE

SEQ ID NO: 18493 - protein, 9 aa, synthetic construct
GGIGIDTLT

SEQ ID NO: 18494 - protein, 9 aa, synthetic construct
GGIGIDTLS

SEQ ID NO: 18495 - protein, 9 aa, synthetic construct
GGIGIDTLN

SEQ ID NO: 18496 - protein, 9 aa, synthetic construct
GGGGPDILK

SEQ ID NO: 18497 - protein, 9 aa, synthetic construct
GGIGIDTFV

SEQ ID NO: 18498 - protein, 9 aa, synthetic construct
GGIGIDTAS

SEQ ID NO: 18499 - protein, 9 aa, synthetic construct
GGIGIDSLT

SEQ ID NO: 18500 - protein, 9 aa, synthetic construct
GGGGPDLII

SEQ ID NO: 18501 - protein, 9 aa, synthetic construct
GGIGIDRLD

SEQ ID NO: 18502 - protein, 9 aa, synthetic construct
GGDGSDAIR

SEQ ID NO: 18503 - protein, 9 aa, synthetic construct
GGDGRDYIA

SEQ ID NO: 18504 - protein, 9 aa, synthetic construct
GGGGNDYVV

SEQ ID NO: 18505 - protein, 9 aa, synthetic construct
GGIGKDSFN

SEQ ID NO: 18506 - protein, 9 aa, synthetic construct
GGIGKDTVS

SEQ ID NO: 18507 - protein, 9 aa, synthetic construct
GGDGRDVLF

SEQ ID NO: 18508 - protein, 9 aa, synthetic construct
GGDGRDVLR

SEQ ID NO: 18509 - protein, 9 aa, synthetic construct
GGDGRDVLV

SEQ ID NO: 18510 - protein, 9 aa, synthetic construct
GGIGKDVLS

SEQ ID NO: 18511 - protein, 9 aa, synthetic construct
GGGGNDYLQ

SEQ ID NO: 18512 - protein, 9 aa, synthetic construct
GGIGKDVFV

SEQ ID NO: 18513 - protein, 9 aa, synthetic construct
GGIGKDTLS

SEQ ID NO: 18514 - protein, 9 aa, synthetic construct
GGGGNDYMV

SEQ ID NO: 18515 - protein, 9 aa, synthetic construct
GGGGNDYLS

SEQ ID NO: 18516 - protein, 9 aa, synthetic construct
GGDGRDVVD

SEQ ID NO: 18517 - protein, 9 aa, synthetic construct
GGDGRDVVR

SEQ ID NO: 18518 - protein, 9 aa, synthetic construct
GGGGNDYLW

SEQ ID NO: 18519 - protein, 9 aa, synthetic construct
GGIGKDTIH

SEQ ID NO: 18520 - protein, 9 aa, synthetic construct
GGGGNDYME

SEQ ID NO: 18521 - protein, 9 aa, synthetic construct
GGDGRDSLV

SEQ ID NO: 18522 - protein, 9 aa, synthetic construct
GGDGRDSLM

SEQ ID NO: 18523 - protein, 9 aa, synthetic construct
GGDGSDALF

SEQ ID NO: 18524 - protein, 9 aa, synthetic construct
GGIGNDSYV

SEQ ID NO: 18525 - protein, 9 aa, synthetic construct
GGIGNDSVQ

SEQ ID NO: 18526 - protein, 9 aa, synthetic construct
GGDGRDMLN

SEQ ID NO: 18527 - protein, 9 aa, synthetic construct
GGDGRDMLT

SEQ ID NO: 18528 - protein, 9 aa, synthetic construct
GGIGNDSMN

SEQ ID NO: 18529 - protein, 9 aa, synthetic construct
GGIGNDSML

SEQ ID NO: 18530 - protein, 9 aa, synthetic construct
GGIGNDSLW

SEQ ID NO: 18531 - protein, 9 aa, synthetic construct
GGIGNDSLR

SEQ ID NO: 18532 - protein, 9 aa, synthetic construct
GGIGNDSLQ

SEQ ID NO: 18533 - protein, 9 aa, synthetic construct
GGIGNDSIL

SEQ ID NO: 18534 - protein, 9 aa, synthetic construct
GGGGNDVMF

SEQ ID NO: 18535 - protein, 9 aa, synthetic construct
GGIGNDSID

SEQ ID NO: 18536 - protein, 9 aa, synthetic construct
GGGGNDVMQ

SEQ ID NO: 18537 - protein, 9 aa, synthetic construct
GGIGNDSFD

SEQ ID NO: 18538 - protein, 9 aa, synthetic construct
GGGGNDVMY

SEQ ID NO: 18539 - protein, 9 aa, synthetic construct
GGGGNDVVE

SEQ ID NO: 18540 - protein, 9 aa, synthetic construct
GGIGNDSVS

SEQ ID NO: 18541 - protein, 9 aa, synthetic construct
GGIGNDTAF

SEQ ID NO: 18542 - protein, 9 aa, synthetic construct
GGDGRDSLL

SEQ ID NO: 18543 - protein, 9 aa, synthetic construct
GGIGNDTAY

SEQ ID NO: 18544 - protein, 9 aa, synthetic construct
GGIGNDTYD

SEQ ID NO: 18545 - protein, 9 aa, synthetic construct
GGDGRDLLL

SEQ ID NO: 18546 - protein, 9 aa, synthetic construct
GGDGRDLLM

SEQ ID NO: 18547 - protein, 9 aa, synthetic construct
GGIGNDTVD

SEQ ID NO: 18548 - protein, 9 aa, synthetic construct
GGIGNDTMV

SEQ ID NO: 18549 - protein, 9 aa, synthetic construct
GGIGNDTMT

SEQ ID NO: 18550 - protein, 9 aa, synthetic construct
GGIGNDTMN

SEQ ID NO: 18551 - protein, 9 aa, synthetic construct
GGIGNDTMD

SEQ ID NO: 18552 - protein, 9 aa, synthetic construct
GGIGNDTMA

SEQ ID NO: 18553 - protein, 9 aa, synthetic construct
GGDGRDLLQ

SEQ ID NO: 18554 - protein, 9 aa, synthetic construct
GGIGNDTIV

SEQ ID NO: 18555 - protein, 9 aa, synthetic construct
GGIGNDTIG

SEQ ID NO: 18556 - protein, 9 aa, synthetic construct
GGIGNDTIE

SEQ ID NO: 18557 - protein, 9 aa, synthetic construct
GGDGRDLVA

SEQ ID NO: 18558 - protein, 9 aa, synthetic construct
GGIGNDTFH

SEQ ID NO: 18559 - protein, 9 aa, synthetic construct
GGIGNDRVD

SEQ ID NO: 18560 - protein, 9 aa, synthetic construct
GGDGRDQLF

SEQ ID NO: 18561 - protein, 9 aa, synthetic construct
GGGGNDVVG

SEQ ID NO: 18562 - protein, 9 aa, synthetic construct
GGDGRDQLL

SEQ ID NO: 18563 - protein, 9 aa, synthetic construct
GGDGRDRVV

SEQ ID NO: 18564 - protein, 9 aa, synthetic construct
GGIGNDLYF

SEQ ID NO: 18565 - protein, 9 aa, synthetic construct
GGIGNDLYA

SEQ ID NO: 18566 - protein, 9 aa, synthetic construct
GGGGNDWLA

SEQ ID NO: 18567 - protein, 9 aa, synthetic construct
GGIGNDLMY

SEQ ID NO: 18568 - protein, 9 aa, synthetic construct
GGIGNDLLY

SEQ ID NO: 18569 - protein, 9 aa, synthetic construct
GGGGNDWLE

SEQ ID NO: 18570 - protein, 9 aa, synthetic construct
GGDGRDSIF

SEQ ID NO: 18571 - protein, 9 aa, synthetic construct
GGIGNDLLL

SEQ ID NO: 18572 - protein, 9 aa, synthetic construct
GGDGRDSIN

SEQ ID NO: 18573 - protein, 9 aa, synthetic construct
GGGGNDWLL

SEQ ID NO: 18574 - protein, 9 aa, synthetic construct
GGDGRDSLA

SEQ ID NO: 18575 - protein, 9 aa, synthetic construct
GGDGRDSLD

SEQ ID NO: 18576 - protein, 9 aa, synthetic construct
GGIGNDLIE

SEQ ID NO: 18577 - protein, 9 aa, synthetic construct
GGGGNDWLN

SEQ ID NO: 18578 - protein, 9 aa, synthetic construct
GGIGNDLYV

SEQ ID NO: 18579 - protein, 9 aa, synthetic construct
GGGGNDWIE

SEQ ID NO: 18580 - protein, 9 aa, synthetic construct
GGGGNDVYY

SEQ ID NO: 18581 - protein, 9 aa, synthetic construct
GGIGNDRIE

SEQ ID NO: 18582 - protein, 9 aa, synthetic construct
GGGGNDVVL

SEQ ID NO: 18583 - protein, 9 aa, synthetic construct
GGIGNDRMH

SEQ ID NO: 18584 - protein, 9 aa, synthetic construct
GGGGNDVVT

SEQ ID NO: 18585 - protein, 9 aa, synthetic construct
GGEGADTLM

SEQ ID NO: 18586 - protein, 9 aa, synthetic construct
GGDGRDRIA

SEQ ID NO: 18587 - protein, 9 aa, synthetic construct
GGIGNDRIG

SEQ ID NO: 18588 - protein, 9 aa, synthetic construct
GGDGRDRIE

SEQ ID NO: 18589 - protein, 9 aa, synthetic construct
GGIGNDMLF

SEQ ID NO: 18590 - protein, 9 aa, synthetic construct
GGGGNDVYK

SEQ ID NO: 18591 - protein, 9 aa, synthetic construct
GGIGNDQLA

SEQ ID NO: 18592 - protein, 9 aa, synthetic construct
GGDGRDRIY

SEQ ID NO: 18593 - protein, 9 aa, synthetic construct
GGIGNDNMG

SEQ ID NO: 18594 - protein, 9 aa, synthetic construct
GGDGRDRLI

SEQ ID NO: 18595 - protein, 9 aa, synthetic construct
GGDGRDRLR

SEQ ID NO: 18596 - protein, 9 aa, synthetic construct
GGDGSDALA

SEQ ID NO: 18597 - protein, 9 aa, synthetic construct
GGDGSDALY

SEQ ID NO: 18598 - protein, 9 aa, synthetic construct
GGIGNDTYW

SEQ ID NO: 18599 - protein, 9 aa, synthetic construct
GGIGDDTLF

SEQ ID NO: 18600 - protein, 9 aa, synthetic construct
GGIGDDTIN

SEQ ID NO: 18601 - protein, 9 aa, synthetic construct
GGDGSDLMD

SEQ ID NO: 18602 - protein, 9 aa, synthetic construct
GGEGADSLI

SEQ ID NO: 18603 - protein, 9 aa, synthetic construct
GGIGDDTFV

SEQ ID NO: 18604 - protein, 9 aa, synthetic construct
GGIGDDTFR

SEQ ID NO: 18605 - protein, 9 aa, synthetic construct
GGIGDDTFI

SEQ ID NO: 18606 - protein, 9 aa, synthetic construct
GGDGSDLMV

SEQ ID NO: 18607 - protein, 9 aa, synthetic construct
GGIGDDSVV

SEQ ID NO: 18608 - protein, 9 aa, synthetic construct
GGGGQDRLV

SEQ ID NO: 18609 - protein, 9 aa, synthetic construct
GGDGSDMAS

SEQ ID NO: 18610 - protein, 9 aa, synthetic construct
GGIGDDSLD

SEQ ID NO: 18611 - protein, 9 aa, synthetic construct
GGDGSDMFV

SEQ ID NO: 18612 - protein, 9 aa, synthetic construct
GGIGDDSID

SEQ ID NO: 18613 - protein, 9 aa, synthetic construct
GGIGDDRYY

SEQ ID NO: 18614 - protein, 9 aa, synthetic construct
GGIGDDRLL

SEQ ID NO: 18615 - protein, 9 aa, synthetic construct
GGIGDDTIV

SEQ ID NO: 18616 - protein, 9 aa, synthetic construct
GGIGDDTLK

SEQ ID NO: 18617 - protein, 9 aa, synthetic construct
GGDGSDLFL

SEQ ID NO: 18618 - protein, 9 aa, synthetic construct
GGIGDDTLW

SEQ ID NO: 18619 - protein, 9 aa, synthetic construct
GGDGSDLID

SEQ ID NO: 18620 - protein, 9 aa, synthetic construct
GGIGDDVVE

SEQ ID NO: 18621 - protein, 9 aa, synthetic construct
GGIGDDVMR

SEQ ID NO: 18622 - protein, 9 aa, synthetic construct
GGDGSDLIE

SEQ ID NO: 18623 - protein, 9 aa, synthetic construct
GGDGSDLIQ

SEQ ID NO: 18624 - protein, 9 aa, synthetic construct
GGIGDDVLE

SEQ ID NO: 18625 - protein, 9 aa, synthetic construct
GGDGSDLIT

SEQ ID NO: 18626 - protein, 9 aa, synthetic construct
GGIGDDVIT

SEQ ID NO: 18627 - protein, 9 aa, synthetic construct
GGIGDDTYT

SEQ ID NO: 18628 - protein, 9 aa, synthetic construct
GGIGDDTYH

SEQ ID NO: 18629 - protein, 9 aa, synthetic construct
GGIGDDTVS

SEQ ID NO: 18630 - protein, 9 aa, synthetic construct
GGIGDDTVG

SEQ ID NO: 18631 - protein, 9 aa, synthetic construct
GGGGQDRIV

SEQ ID NO: 18632 - protein, 9 aa, synthetic construct
GGIGDDTMF

SEQ ID NO: 18633 - protein, 9 aa, synthetic construct
GGIGDDTME

SEQ ID NO: 18634 - protein, 9 aa, synthetic construct
GGGGQDSLS

SEQ ID NO: 18635 - protein, 9 aa, synthetic construct
GGIGDDRIY

SEQ ID NO: 18636 - protein, 9 aa, synthetic construct
GGIGDDRIE

SEQ ID NO: 18637 - protein, 9 aa, synthetic construct
GGIGDDRID

SEQ ID NO: 18638 - protein, 9 aa, synthetic construct
GGIGDDIYL

SEQ ID NO: 18639 - protein, 9 aa, synthetic construct
GGDGSDRFV

SEQ ID NO: 18640 - protein, 9 aa, synthetic construct
GGEGADRMV

SEQ ID NO: 18641 - protein, 9 aa, synthetic construct
GGIGDDIVG

SEQ ID NO: 18642 - protein, 9 aa, synthetic construct
GGIGDDIMT

SEQ ID NO: 18643 - protein, 9 aa, synthetic construct
GGDGSDRIY

SEQ ID NO: 18644 - protein, 9 aa, synthetic construct
GGDGSDRLA

SEQ ID NO: 18645 - protein, 9 aa, synthetic construct
GGIGDDILN

SEQ ID NO: 18646 - protein, 9 aa, synthetic construct
GGIGDDILF

SEQ ID NO: 18647 - protein, 9 aa, synthetic construct
GGIGDDIIY

SEQ ID NO: 18648 - protein, 9 aa, synthetic construct
GGIGDDIIW

SEQ ID NO: 18649 - protein, 9 aa, synthetic construct
GGIGDDIIT

SEQ ID NO: 18650 - protein, 9 aa, synthetic construct
GGDGSDRLE

SEQ ID NO: 18651 - protein, 9 aa, synthetic construct
GGIGDDIIC

SEQ ID NO: 18652 - protein, 9 aa, synthetic construct
GGDGSDRLI

SEQ ID NO: 18653 - protein, 9 aa, synthetic construct
GGGGQDTLL

SEQ ID NO: 18654 - protein, 9 aa, synthetic construct
GGDGSDQVT

SEQ ID NO: 18655 - protein, 9 aa, synthetic construct
GGIGDDLII

SEQ ID NO: 18656 - protein, 9 aa, synthetic construct
GGIGDDNLM

SEQ ID NO: 18657 - protein, 9 aa, synthetic construct
GGDGSDNIN

SEQ ID NO: 18658 - protein, 9 aa, synthetic construct
GGGGQDSLY

SEQ ID NO: 18659 - protein, 9 aa, synthetic construct
GGDGSDNLA

SEQ ID NO: 18660 - protein, 9 aa, synthetic construct
GGEGADSID

SEQ ID NO: 18661 - protein, 9 aa, synthetic construct
GGIGDDNVN

SEQ ID NO: 18662 - protein, 9 aa, synthetic construct
GGIGDDNLN

SEQ ID NO: 18663 - protein, 9 aa, synthetic construct
GGIGDDNLD

SEQ ID NO: 18664 - protein, 9 aa, synthetic construct
GGIGDDLIQ

SEQ ID NO: 18665 - protein, 9 aa, synthetic construct
GGEGADSFV

SEQ ID NO: 18666 - protein, 9 aa, synthetic construct
GGDGSDQLD

SEQ ID NO: 18667 - protein, 9 aa, synthetic construct
GGIGDDLLY

SEQ ID NO: 18668 - protein, 9 aa, synthetic construct
GGIGDDLLT

SEQ ID NO: 18669 - protein, 9 aa, synthetic construct
GGIGDDLLR

SEQ ID NO: 18670 - protein, 9 aa, synthetic construct
GGIGDDLLA

SEQ ID NO: 18671 - protein, 9 aa, synthetic construct
GGIGDDVYF

SEQ ID NO: 18672 - protein, 9 aa, synthetic construct
GGIGDDWLY

SEQ ID NO: 18673 - protein, 9 aa, synthetic construct
GGEGADTFS

SEQ ID NO: 18674 - protein, 9 aa, synthetic construct
GGGGQDEMT

SEQ ID NO: 18675 - protein, 9 aa, synthetic construct
GGGGQDFIN

SEQ ID NO: 18676 - protein, 9 aa, synthetic construct
GGEGADTAD

SEQ ID NO: 18677 - protein, 9 aa, synthetic construct
GGDGSDFLY

SEQ ID NO: 18678 - protein, 9 aa, synthetic construct
GGGGQDHLR

SEQ ID NO: 18679 - protein, 9 aa, synthetic construct
GGIGGDTYI

SEQ ID NO: 18680 - protein, 9 aa, synthetic construct
GGDGSDFVA

SEQ ID NO: 18681 - protein, 9 aa, synthetic construct
GGIGGDTLT

SEQ ID NO: 18682 - protein, 9 aa, synthetic construct
GGIGGDTLN

SEQ ID NO: 18683 - protein, 9 aa, synthetic construct
GGGGQDIID

SEQ ID NO: 18684 - protein, 9 aa, synthetic construct
GGIGGDSME

SEQ ID NO: 18685 - protein, 9 aa, synthetic construct
GGIGGDSLS

SEQ ID NO: 18686 - protein, 9 aa, synthetic construct
GGIGGDSIS

SEQ ID NO: 18687 - protein, 9 aa, synthetic construct
GGDGSDFYY

SEQ ID NO: 18688 - protein, 9 aa, synthetic construct
GGDGSDGIS

SEQ ID NO: 18689 - protein, 9 aa, synthetic construct
GGIGGDRLV

SEQ ID NO: 18690 - protein, 9 aa, synthetic construct
GGDGSDFLL

SEQ ID NO: 18691 - protein, 9 aa, synthetic construct
GGGGQDELT

SEQ ID NO: 18692 - protein, 9 aa, synthetic construct
GGIGDDYID

SEQ ID NO: 18693 - protein, 9 aa, synthetic construct
GGGGQDDLY

SEQ ID NO: 18694 - protein, 9 aa, synthetic construct
GGDGSDAYH

SEQ ID NO: 18695 - protein, 9 aa, synthetic construct
GGGGPDRLE

SEQ ID NO: 18696 - protein, 9 aa, synthetic construct
GGDGSDDLT

SEQ ID NO: 18697 - protein, 9 aa, synthetic construct
GGIGHDTYV

SEQ ID NO: 18698 - protein, 9 aa, synthetic construct
GGDGSDDLY

SEQ ID NO: 18699 - protein, 9 aa, synthetic construct
GGIGHDTLR

SEQ ID NO: 18700 - protein, 9 aa, synthetic construct
GGGGPDTLR

SEQ ID NO: 18701 - protein, 9 aa, synthetic construct
GGDGSDELF

SEQ ID NO: 18702 - protein, 9 aa, synthetic construct
GGEGADTFA

SEQ ID NO: 18703 - protein, 9 aa, synthetic construct
GGDGSDELS

SEQ ID NO: 18704 - protein, 9 aa, synthetic construct
GGGGQDAFV

SEQ ID NO: 18705 - protein, 9 aa, synthetic construct
GGIGHDLVT

SEQ ID NO: 18706 - protein, 9 aa, synthetic construct
GGDGSDELW

SEQ ID NO: 18707 - protein, 9 aa, synthetic construct
GGGGQDALF

SEQ ID NO: 18708 - protein, 9 aa, synthetic construct
GGGGQDDLS

SEQ ID NO: 18709 - protein, 9 aa, synthetic construct
GGIGGDRLD

SEQ ID NO: 18710 - protein, 9 aa, synthetic construct
GGIGGDRFI

SEQ ID NO: 18711 - protein, 9 aa, synthetic construct
GGEGADSVD

SEQ ID NO: 18712 - protein, 9 aa, synthetic construct
GGDGSDGLY

SEQ ID NO: 18713 - protein, 9 aa, synthetic construct
GGIGFDLLR

SEQ ID NO: 18714 - protein, 9 aa, synthetic construct
GGGGQDLLQ

SEQ ID NO: 18715 - protein, 9 aa, synthetic construct
GGGGQDLLS

SEQ ID NO: 18716 - protein, 9 aa, synthetic construct
GGIGEDVVQ

SEQ ID NO: 18717 - protein, 9 aa, synthetic construct
GGGGQDLLV

SEQ ID NO: 18718 - protein, 9 aa, synthetic construct
GGIGEDVIL

SEQ ID NO: 18719 - protein, 9 aa, synthetic construct
GGDGSDIVD

SEQ ID NO: 18720 - protein, 9 aa, synthetic construct
GGDGSDIVQ

SEQ ID NO: 18721 - protein, 9 aa, synthetic construct
GGDGSDIYL

SEQ ID NO: 18722 - protein, 9 aa, synthetic construct
GGIGEDSLY

SEQ ID NO: 18723 - protein, 9 aa, synthetic construct
GGEGADSLT

SEQ ID NO: 18724 - protein, 9 aa, synthetic construct
GGEGADSLN

SEQ ID NO: 18725 - protein, 9 aa, synthetic construct
GGIGEDAIL

SEQ ID NO: 18726 - protein, 9 aa, synthetic construct
GGIGDDYLE

SEQ ID NO: 18727 - protein, 9 aa, synthetic construct
GGIGDDYLD

SEQ ID NO: 18728 - protein, 9 aa, synthetic construct
GGIGFDLLV

SEQ ID NO: 18729 - protein, 9 aa, synthetic construct
GGIGFDRLT

SEQ ID NO: 18730 - protein, 9 aa, synthetic construct
GGIGFDSAD

SEQ ID NO: 18731 - protein, 9 aa, synthetic construct
GGEGADSMQ

SEQ ID NO: 18732 - protein, 9 aa, synthetic construct
GGDGSDGVD

SEQ ID NO: 18733 - protein, 9 aa, synthetic construct
GGIGGDLMY

SEQ ID NO: 18734 - protein, 9 aa, synthetic construct
GGIGGDLLD

SEQ ID NO: 18735 - protein, 9 aa, synthetic construct
GGEGADSMT

SEQ ID NO: 18736 - protein, 9 aa, synthetic construct
GGDGSDIFL

SEQ ID NO: 18737 - protein, 9 aa, synthetic construct
GGIGGDALD

SEQ ID NO: 18738 - protein, 9 aa, synthetic construct
GGIGFDTLS

SEQ ID NO: 18739 - protein, 9 aa, synthetic construct
GGDGSDILA

SEQ ID NO: 18740 - protein, 9 aa, synthetic construct
GGIGFDTLL

SEQ ID NO: 18741 - protein, 9 aa, synthetic construct
GGIGFDTLA

SEQ ID NO: 18742 - protein, 9 aa, synthetic construct
GGDGSDIIS

SEQ ID NO: 18743 - protein, 9 aa, synthetic construct
GGDGSDIIV

SEQ ID NO: 18744 - protein, 9 aa, synthetic construct
GGIGFDTAS

SEQ ID NO: 18745 - protein, 9 aa, synthetic construct
GGIGFDTAD

SEQ ID NO: 18746 - protein, 9 aa, synthetic construct
GGIGNDTYK

SEQ ID NO: 18747 - protein, 9 aa, synthetic construct
GGIGNDVFA

SEQ ID NO: 18748 - protein, 9 aa, synthetic construct
GGDGNDWIS

SEQ ID NO: 18749 - protein, 9 aa, synthetic construct
GGKGADLLH

SEQ ID NO: 18750 - protein, 9 aa, synthetic construct
GGKGADLIY

SEQ ID NO: 18751 - protein, 9 aa, synthetic construct
GGDGPDSLI

SEQ ID NO: 18752 - protein, 9 aa, synthetic construct
GGDGPDTFI

SEQ ID NO: 18753 - protein, 9 aa, synthetic construct
GGKGADLFV

SEQ ID NO: 18754 - protein, 9 aa, synthetic construct
GGKGADKMT

SEQ ID NO: 18755 - protein, 9 aa, synthetic construct
GGKGADKLW

SEQ ID NO: 18756 - protein, 9 aa, synthetic construct
GGKGADKLF

SEQ ID NO: 18757 - protein, 9 aa, synthetic construct
GGDGPDTIN

SEQ ID NO: 18758 - protein, 9 aa, synthetic construct
GGKGADIVV

SEQ ID NO: 18759 - protein, 9 aa, synthetic construct
GGKGADIMR

SEQ ID NO: 18760 - protein, 9 aa, synthetic construct
GGDGPDTLL

SEQ ID NO: 18761 - protein, 9 aa, synthetic construct
GGEGADVFF

SEQ ID NO: 18762 - protein, 9 aa, synthetic construct
GGKGADILY

SEQ ID NO: 18763 - protein, 9 aa, synthetic construct
GGKGADILS

SEQ ID NO: 18764 - protein, 9 aa, synthetic construct
GGKGADILR

SEQ ID NO: 18765 - protein, 9 aa, synthetic construct
GGKGADLLA

SEQ ID NO: 18766 - protein, 9 aa, synthetic construct
GGDGPDRLS

SEQ ID NO: 18767 - protein, 9 aa, synthetic construct
GGKGADRLT

SEQ ID NO: 18768 - protein, 9 aa, synthetic construct
GGGGNDSIT

SEQ ID NO: 18769 - protein, 9 aa, synthetic construct
GGKGADRLA

SEQ ID NO: 18770 - protein, 9 aa, synthetic construct
GGKGADRIT

SEQ ID NO: 18771 - protein, 9 aa, synthetic construct
GGKGADRFM

SEQ ID NO: 18772 - protein, 9 aa, synthetic construct
GGKGADQMT

SEQ ID NO: 18773 - protein, 9 aa, synthetic construct
GGGGNDSFV

SEQ ID NO: 18774 - protein, 9 aa, synthetic construct
GGGGNDSFW

SEQ ID NO: 18775 - protein, 9 aa, synthetic construct
GGKGADQIT

SEQ ID NO: 18776 - protein, 9 aa, synthetic construct
GGKGADQIS

SEQ ID NO: 18777 - protein, 9 aa, synthetic construct
GGDGPDNIV

SEQ ID NO: 18778 - protein, 9 aa, synthetic construct
GGKGADNLI

SEQ ID NO: 18779 - protein, 9 aa, synthetic construct
GGKGADMLV

SEQ ID NO: 18780 - protein, 9 aa, synthetic construct
GGKGADMLL

SEQ ID NO: 18781 - protein, 9 aa, synthetic construct
GGKGADMLD

SEQ ID NO: 18782 - protein, 9 aa, synthetic construct
GGKGADLLV

SEQ ID NO: 18783 - protein, 9 aa, synthetic construct
GGKGADLLT

SEQ ID NO: 18784 - protein, 9 aa, synthetic construct
GGKGADILA

SEQ ID NO: 18785 - protein, 9 aa, synthetic construct
GGKGADIIY

SEQ ID NO: 18786 - protein, 9 aa, synthetic construct
GGKGADIID

SEQ ID NO: 18787 - protein, 9 aa, synthetic construct
GGKGADIFV

SEQ ID NO: 18788 - protein, 9 aa, synthetic construct
GGKGADDLN

SEQ ID NO: 18789 - protein, 9 aa, synthetic construct
GGKGADDLD

SEQ ID NO: 18790 - protein, 9 aa, synthetic construct
GGDGQDFIV

SEQ ID NO: 18791 - protein, 9 aa, synthetic construct
GGDGQDFLF

SEQ ID NO: 18792 - protein, 9 aa, synthetic construct
GGDGQDFLI

SEQ ID NO: 18793 - protein, 9 aa, synthetic construct
GGDGQDFLY

SEQ ID NO: 18794 - protein, 9 aa, synthetic construct
GGKGADALK

SEQ ID NO: 18795 - protein, 9 aa, synthetic construct
GGDGQDFMT

SEQ ID NO: 18796 - protein, 9 aa, synthetic construct
GGEGADTVT

SEQ ID NO: 18797 - protein, 9 aa, synthetic construct
GGDGQDGLY

SEQ ID NO: 18798 - protein, 9 aa, synthetic construct
GGDGQDHLM

SEQ ID NO: 18799 - protein, 9 aa, synthetic construct
GGIGYDSLY

SEQ ID NO: 18800 - protein, 9 aa, synthetic construct
GGIGYDRLT

SEQ ID NO: 18801 - protein, 9 aa, synthetic construct
GGIGYDIYV

SEQ ID NO: 18802 - protein, 9 aa, synthetic construct
GGIGYDILN

SEQ ID NO: 18803 - protein, 9 aa, synthetic construct
GGKGADDLT

SEQ ID NO: 18804 - protein, 9 aa, synthetic construct
GGKGADELD

SEQ ID NO: 18805 - protein, 9 aa, synthetic construct
GGEGADTYH

SEQ ID NO: 18806 - protein, 9 aa, synthetic construct
GGKGADGLL

SEQ ID NO: 18807 - protein, 9 aa, synthetic construct
GGKGADIFL

SEQ ID NO: 18808 - protein, 9 aa, synthetic construct
GGDGPDVLD

SEQ ID NO: 18809 - protein, 9 aa, synthetic construct
GGKGADHMD

SEQ ID NO: 18810 - protein, 9 aa, synthetic construct
GGDGPDVLS

SEQ ID NO: 18811 - protein, 9 aa, synthetic construct
GGKGADHFY

SEQ ID NO: 18812 - protein, 9 aa, synthetic construct
GGGGNDSLQ

SEQ ID NO: 18813 - protein, 9 aa, synthetic construct
GGDGPDYFV

SEQ ID NO: 18814 - protein, 9 aa, synthetic construct
GGGGNDSVD

SEQ ID NO: 18815 - protein, 9 aa, synthetic construct
GGKGADFLT

SEQ ID NO: 18816 - protein, 9 aa, synthetic construct
GGDGQDALN

SEQ ID NO: 18817 - protein, 9 aa, synthetic construct
GGKGADEVD

SEQ ID NO: 18818 - protein, 9 aa, synthetic construct
GGKGADEMY

SEQ ID NO: 18819 - protein, 9 aa, synthetic construct
GGEGADTYR

SEQ ID NO: 18820 - protein, 9 aa, synthetic construct
GGKGADELH

SEQ ID NO: 18821 - protein, 9 aa, synthetic construct
GGKGADRLF

SEQ ID NO: 18822 - protein, 9 aa, synthetic construct
GGKGADRLY

SEQ ID NO: 18823 - protein, 9 aa, synthetic construct
GGIGWDEIH

SEQ ID NO: 18824 - protein, 9 aa, synthetic construct
GGDGNDWMS

SEQ ID NO: 18825 - protein, 9 aa, synthetic construct
GGDGNDWVD

SEQ ID NO: 18826 - protein, 9 aa, synthetic construct
GGEGADVIR

SEQ ID NO: 18827 - protein, 9 aa, synthetic construct
GGKGDDDIR

SEQ ID NO: 18828 - protein, 9 aa, synthetic construct
GGDGNDYAF

SEQ ID NO: 18829 - protein, 9 aa, synthetic construct
GGGGNDRML

SEQ ID NO: 18830 - protein, 9 aa, synthetic construct
GGKGDDALR

SEQ ID NO: 18831 - protein, 9 aa, synthetic construct
GGDGNDYIA

SEQ ID NO: 18832 - protein, 9 aa, synthetic construct
GGKGCDTLT

SEQ ID NO: 18833 - protein, 9 aa, synthetic construct
GGGGNDRVF

SEQ ID NO: 18834 - protein, 9 aa, synthetic construct
GGEGADVIL

SEQ ID NO: 18835 - protein, 9 aa, synthetic construct
GGKGADYLD

SEQ ID NO: 18836 - protein, 9 aa, synthetic construct
GGGGNDRVV

SEQ ID NO: 18837 - protein, 9 aa, synthetic construct
GGKGADWIS

SEQ ID NO: 18838 - protein, 9 aa, synthetic construct
GGKGADWIN

SEQ ID NO: 18839 - protein, 9 aa, synthetic construct
GGDGNDYIS

SEQ ID NO: 18840 - protein, 9 aa, synthetic construct
GGGGNDRMD

SEQ ID NO: 18841 - protein, 9 aa, synthetic construct
GGKGDDEIG

SEQ ID NO: 18842 - protein, 9 aa, synthetic construct
GGDGPDHLT

SEQ ID NO: 18843 - protein, 9 aa, synthetic construct
GGKGDDEII

SEQ ID NO: 18844 - protein, 9 aa, synthetic construct
GGDGNDWIY

SEQ ID NO: 18845 - protein, 9 aa, synthetic construct
GGKGDDHLI

SEQ ID NO: 18846 - protein, 9 aa, synthetic construct
GGKGDDFVT

SEQ ID NO: 18847 - protein, 9 aa, synthetic construct
GGDGNDWLI

SEQ ID NO: 18848 - protein, 9 aa, synthetic construct
GGKGDDFLY

SEQ ID NO: 18849 - protein, 9 aa, synthetic construct
GGKGDDFLI

SEQ ID NO: 18850 - protein, 9 aa, synthetic construct
GGKGDDFLD

SEQ ID NO: 18851 - protein, 9 aa, synthetic construct
GGDGNDWLL

SEQ ID NO: 18852 - protein, 9 aa, synthetic construct
GGKGDDFIV

SEQ ID NO: 18853 - protein, 9 aa, synthetic construct
GGKGDDELT

SEQ ID NO: 18854 - protein, 9 aa, synthetic construct
GGKGDDELR

SEQ ID NO: 18855 - protein, 9 aa, synthetic construct
GGKGDDELQ

SEQ ID NO: 18856 - protein, 9 aa, synthetic construct
GGKGDDELH

SEQ ID NO: 18857 - protein, 9 aa, synthetic construct
GGDGNDWMD

SEQ ID NO: 18858 - protein, 9 aa, synthetic construct
GGKGDDEIR

SEQ ID NO: 18859 - protein, 9 aa, synthetic construct
GGKGADVME

SEQ ID NO: 18860 - protein, 9 aa, synthetic construct
GGDGNDYIT

SEQ ID NO: 18861 - protein, 9 aa, synthetic construct
GGKGADVLN

SEQ ID NO: 18862 - protein, 9 aa, synthetic construct
GGKGADVLD

SEQ ID NO: 18863 - protein, 9 aa, synthetic construct
GGKGADTFA

SEQ ID NO: 18864 - protein, 9 aa, synthetic construct
GGKGADTAT

SEQ ID NO: 18865 - protein, 9 aa, synthetic construct
GGDGNDYVK

SEQ ID NO: 18866 - protein, 9 aa, synthetic construct
GGKGADTAI

SEQ ID NO: 18867 - protein, 9 aa, synthetic construct
GGGGNDRYG

SEQ ID NO: 18868 - protein, 9 aa, synthetic construct
GGKGADSLV

SEQ ID NO: 18869 - protein, 9 aa, synthetic construct
GGGGNDRYM

SEQ ID NO: 18870 - protein, 9 aa, synthetic construct
GGKGADSLF

SEQ ID NO: 18871 - protein, 9 aa, synthetic construct
GGKGADSLD

SEQ ID NO: 18872 - protein, 9 aa, synthetic construct
GGKGADSIF

SEQ ID NO: 18873 - protein, 9 aa, synthetic construct
GGKGADSIE

SEQ ID NO: 18874 - protein, 9 aa, synthetic construct
GGGGNDRYV

SEQ ID NO: 18875 - protein, 9 aa, synthetic construct
GGKGADSFI

SEQ ID NO: 18876 - protein, 9 aa, synthetic construct
GGGGNDSAA

SEQ ID NO: 18877 - protein, 9 aa, synthetic construct
GGKGADSFE

SEQ ID NO: 18878 - protein, 9 aa, synthetic construct
GGKGADTFR

SEQ ID NO: 18879 - protein, 9 aa, synthetic construct
GGKGADTIA

SEQ ID NO: 18880 - protein, 9 aa, synthetic construct
GGDGNDYMV

SEQ ID NO: 18881 - protein, 9 aa, synthetic construct
GGDGNDYLQ

SEQ ID NO: 18882 - protein, 9 aa, synthetic construct
GGDGNDYLC

SEQ ID NO: 18883 - protein, 9 aa, synthetic construct
GGKGADVFT

SEQ ID NO: 18884 - protein, 9 aa, synthetic construct
GGKGADVFK

SEQ ID NO: 18885 - protein, 9 aa, synthetic construct
GGKGADVFF

SEQ ID NO: 18886 - protein, 9 aa, synthetic construct
GGKGADTYQ

SEQ ID NO: 18887 - protein, 9 aa, synthetic construct
GGDGNDYLM

SEQ ID NO: 18888 - protein, 9 aa, synthetic construct
GGDGNDYLW

SEQ ID NO: 18889 - protein, 9 aa, synthetic construct
GGKGADTIG

SEQ ID NO: 18890 - protein, 9 aa, synthetic construct
GGKGADTLH

SEQ ID NO: 18891 - protein, 9 aa, synthetic construct
GGDGNDYMG

SEQ ID NO: 18892 - protein, 9 aa, synthetic construct
GGKGADTLA

SEQ ID NO: 18893 - protein, 9 aa, synthetic construct
GGKGADTIV

SEQ ID NO: 18894 - protein, 9 aa, synthetic construct
GGKGADTIS

SEQ ID NO: 18895 - protein, 9 aa, synthetic construct
GGKGADTIK

SEQ ID NO: 18896 - protein, 9 aa, synthetic construct
GGIGYDDIY

SEQ ID NO: 18897 - protein, 9 aa, synthetic construct
GGDGQDIFS

SEQ ID NO: 18898 - protein, 9 aa, synthetic construct
GGIGNDVFY

SEQ ID NO: 18899 - protein, 9 aa, synthetic construct
GGIGRDRLI

SEQ ID NO: 18900 - protein, 9 aa, synthetic construct
GGIGRDRLD

SEQ ID NO: 18901 - protein, 9 aa, synthetic construct
GGDGRDDIF

SEQ ID NO: 18902 - protein, 9 aa, synthetic construct
GGGGNDTYR

SEQ ID NO: 18903 - protein, 9 aa, synthetic construct
GGEGADTMY

SEQ ID NO: 18904 - protein, 9 aa, synthetic construct
GGGGNDTYW

SEQ ID NO: 18905 - protein, 9 aa, synthetic construct
GGIGRDMLH

SEQ ID NO: 18906 - protein, 9 aa, synthetic construct
GGIGRDLII

SEQ ID NO: 18907 - protein, 9 aa, synthetic construct
GGDGRDDLN

SEQ ID NO: 18908 - protein, 9 aa, synthetic construct
GGIGRDKLV

SEQ ID NO: 18909 - protein, 9 aa, synthetic construct
GGDGRDEAH

SEQ ID NO: 18910 - protein, 9 aa, synthetic construct
GGDGRDEIL

SEQ ID NO: 18911 - protein, 9 aa, synthetic construct
GGIGRDIMT

SEQ ID NO: 18912 - protein, 9 aa, synthetic construct
GGDGRDEIV

SEQ ID NO: 18913 - protein, 9 aa, synthetic construct
GGIGRDIIY

SEQ ID NO: 18914 - protein, 9 aa, synthetic construct
GGGGNDVAV

SEQ ID NO: 18915 - protein, 9 aa, synthetic construct
GGDGRDCLD

SEQ ID NO: 18916 - protein, 9 aa, synthetic construct
GGIGRDSIQ

SEQ ID NO: 18917 - protein, 9 aa, synthetic construct
GGIGSDDLA

SEQ ID NO: 18918 - protein, 9 aa, synthetic construct
GGDGRDAMA

SEQ ID NO: 18919 - protein, 9 aa, synthetic construct
GGGGNDTMW

SEQ ID NO: 18920 - protein, 9 aa, synthetic construct
GGDGQDVMS

SEQ ID NO: 18921 - protein, 9 aa, synthetic construct
GGIGRDVLS

SEQ ID NO: 18922 - protein, 9 aa, synthetic construct
GGDGQDYLD

SEQ ID NO: 18923 - protein, 9 aa, synthetic construct
GGDGQDYLE

SEQ ID NO: 18924 - protein, 9 aa, synthetic construct
GGDGQDYLS

SEQ ID NO: 18925 - protein, 9 aa, synthetic construct
GGIGRDVFY

SEQ ID NO: 18926 - protein, 9 aa, synthetic construct
GGGGNDTVH

SEQ ID NO: 18927 - protein, 9 aa, synthetic construct
GGIGRDTMR

SEQ ID NO: 18928 - protein, 9 aa, synthetic construct
GGIGRDTLI

SEQ ID NO: 18929 - protein, 9 aa, synthetic construct
GGIGRDTLF

SEQ ID NO: 18930 - protein, 9 aa, synthetic construct
GGIGRDTLE

SEQ ID NO: 18931 - protein, 9 aa, synthetic construct
GGIGRDTIN

SEQ ID NO: 18932 - protein, 9 aa, synthetic construct
GGIGRDSLV

SEQ ID NO: 18933 - protein, 9 aa, synthetic construct
GGIGRDSLN

SEQ ID NO: 18934 - protein, 9 aa, synthetic construct
GGIGQDYLN

SEQ ID NO: 18935 - protein, 9 aa, synthetic construct
GGIGQDYLD

SEQ ID NO: 18936 - protein, 9 aa, synthetic construct
GGDGRDELY

SEQ ID NO: 18937 - protein, 9 aa, synthetic construct
GGDGRDEMQ

SEQ ID NO: 18938 - protein, 9 aa, synthetic construct
GGIGNDWLI

SEQ ID NO: 18939 - protein, 9 aa, synthetic construct
GGGGNDVIK

SEQ ID NO: 18940 - protein, 9 aa, synthetic construct
GGDGRDKLD

SEQ ID NO: 18941 - protein, 9 aa, synthetic construct
GGDGRDKLF

SEQ ID NO: 18942 - protein, 9 aa, synthetic construct
GGIGNDVYI

SEQ ID NO: 18943 - protein, 9 aa, synthetic construct
GGDGRDKLM

SEQ ID NO: 18944 - protein, 9 aa, synthetic construct
GGDGRDKLS

SEQ ID NO: 18945 - protein, 9 aa, synthetic construct
GGDGRDKLY

SEQ ID NO: 18946 - protein, 9 aa, synthetic construct
GGDGRDKVF

SEQ ID NO: 18947 - protein, 9 aa, synthetic construct
GGIGNDVMD

SEQ ID NO: 18948 - protein, 9 aa, synthetic construct
GGIGNDVLW

SEQ ID NO: 18949 - protein, 9 aa, synthetic construct
GGIGNDVLM

SEQ ID NO: 18950 - protein, 9 aa, synthetic construct
GGIGNDVIT

SEQ ID NO: 18951 - protein, 9 aa, synthetic construct
GGDGRDLFV

SEQ ID NO: 18952 - protein, 9 aa, synthetic construct
GGIGNDVIF

SEQ ID NO: 18953 - protein, 9 aa, synthetic construct
GGIGNDWLS

SEQ ID NO: 18954 - protein, 9 aa, synthetic construct
GGIGNDYIS

SEQ ID NO: 18955 - protein, 9 aa, synthetic construct
GGDGRDKAW

SEQ ID NO: 18956 - protein, 9 aa, synthetic construct
GGDGRDIAS

SEQ ID NO: 18957 - protein, 9 aa, synthetic construct
GGIGQDTMR

SEQ ID NO: 18958 - protein, 9 aa, synthetic construct
GGIGQDTIF

SEQ ID NO: 18959 - protein, 9 aa, synthetic construct
GGIGQDSLF

SEQ ID NO: 18960 - protein, 9 aa, synthetic construct
GGGGNDVFQ

SEQ ID NO: 18961 - protein, 9 aa, synthetic construct
GGIGQDMLF

SEQ ID NO: 18962 - protein, 9 aa, synthetic construct
GGIGQDLLH

SEQ ID NO: 18963 - protein, 9 aa, synthetic construct
GGDGRDIFV

SEQ ID NO: 18964 - protein, 9 aa, synthetic construct
GGIGNDYLT

SEQ ID NO: 18965 - protein, 9 aa, synthetic construct
GGDGRDILI

SEQ ID NO: 18966 - protein, 9 aa, synthetic construct
GGDGRDILS

SEQ ID NO: 18967 - protein, 9 aa, synthetic construct
GGGGNDVIE

SEQ ID NO: 18968 - protein, 9 aa, synthetic construct
GGIGPDLLK

SEQ ID NO: 18969 - protein, 9 aa, synthetic construct
GGDGRDIVL

SEQ ID NO: 18970 - protein, 9 aa, synthetic construct
GGIGPDALM

SEQ ID NO: 18971 - protein, 9 aa, synthetic construct
GGGGNDTMV

SEQ ID NO: 18972 - protein, 9 aa, synthetic construct
GGGGNDTMR

SEQ ID NO: 18973 - protein, 9 aa, synthetic construct
GGIGWDDIF

SEQ ID NO: 18974 - protein, 9 aa, synthetic construct
GGIGTDVFV

SEQ ID NO: 18975 - protein, 9 aa, synthetic construct
GGIGTDTLS

SEQ ID NO: 18976 - protein, 9 aa, synthetic construct
GGIGTDTLL

SEQ ID NO: 18977 - protein, 9 aa, synthetic construct
GGDGQDNLN

SEQ ID NO: 18978 - protein, 9 aa, synthetic construct
GGIGTDTIN

SEQ ID NO: 18979 - protein, 9 aa, synthetic construct
GGIGTDTAV

SEQ ID NO: 18980 - protein, 9 aa, synthetic construct
GGDGQDQIS

SEQ ID NO: 18981 - protein, 9 aa, synthetic construct
GGIGTDSLT

SEQ ID NO: 18982 - protein, 9 aa, synthetic construct
GGIGTDKLF

SEQ ID NO: 18983 - protein, 9 aa, synthetic construct
GGIGTDILI

SEQ ID NO: 18984 - protein, 9 aa, synthetic construct
GGIGTDHLS

SEQ ID NO: 18985 - protein, 9 aa, synthetic construct
GGIGTDFLY

SEQ ID NO: 18986 - protein, 9 aa, synthetic construct
GGDGQDRLL

SEQ ID NO: 18987 - protein, 9 aa, synthetic construct
GGDGQDRLR

SEQ ID NO: 18988 - protein, 9 aa, synthetic construct
GGIGSDWLY

SEQ ID NO: 18989 - protein, 9 aa, synthetic construct
GGIGSDVLV

SEQ ID NO: 18990 - protein, 9 aa, synthetic construct
GGIGTDTVD

SEQ ID NO: 18991 - protein, 9 aa, synthetic construct
GGIGTDVLI

SEQ ID NO: 18992 - protein, 9 aa, synthetic construct
GGGGNDTMK

SEQ ID NO: 18993 - protein, 9 aa, synthetic construct
GGIGTDVLN

SEQ ID NO: 18994 - protein, 9 aa, synthetic construct
GGIGVDYLA

SEQ ID NO: 18995 - protein, 9 aa, synthetic construct
GGGGNDTAV

SEQ ID NO: 18996 - protein, 9 aa, synthetic construct
GGDGQDIIR

SEQ ID NO: 18997 - protein, 9 aa, synthetic construct
GGDGQDILD

SEQ ID NO: 18998 - protein, 9 aa, synthetic construct
GGIGVDTYA

SEQ ID NO: 18999 - protein, 9 aa, synthetic construct
GGDGQDIVH

SEQ ID NO: 19000 - protein, 9 aa, synthetic construct
GGEGADTVN

SEQ ID NO: 19001 - protein, 9 aa, synthetic construct
GGIGVDSMA

SEQ ID NO: 19002 - protein, 9 aa, synthetic construct
GGIGVDRVE

SEQ ID NO: 19003 - protein, 9 aa, synthetic construct
GGDGQDLIA

SEQ ID NO: 19004 - protein, 9 aa, synthetic construct
GGIGVDLMT

SEQ ID NO: 19005 - protein, 9 aa, synthetic construct
GGGGNDTFQ

SEQ ID NO: 19006 - protein, 9 aa, synthetic construct
GGIGVDKMI

SEQ ID NO: 19007 - protein, 9 aa, synthetic construct
GGIGVDILS

SEQ ID NO: 19008 - protein, 9 aa, synthetic construct
GGDGQDLLL

SEQ ID NO: 19009 - protein, 9 aa, synthetic construct
GGIGSDVLS

SEQ ID NO: 19010 - protein, 9 aa, synthetic construct
GGDGQDRLY

SEQ ID NO: 19011 - protein, 9 aa, synthetic construct
GGIGSDVIL

SEQ ID NO: 19012 - protein, 9 aa, synthetic construct
GGDGQDSLA

SEQ ID NO: 19013 - protein, 9 aa, synthetic construct
GGDGQDTLA

SEQ ID NO: 19014 - protein, 9 aa, synthetic construct
GGIGSDQLE

SEQ ID NO: 19015 - protein, 9 aa, synthetic construct
GGIGSDQLD

SEQ ID NO: 19016 - protein, 9 aa, synthetic construct
GGDGQDTLN

SEQ ID NO: 19017 - protein, 9 aa, synthetic construct
GGIGSDLLS

SEQ ID NO: 19018 - protein, 9 aa, synthetic construct
GGDGQDTLT

SEQ ID NO: 19019 - protein, 9 aa, synthetic construct
GGDGQDTLV

SEQ ID NO: 19020 - protein, 9 aa, synthetic construct
GGIGSDKLI

SEQ ID NO: 19021 - protein, 9 aa, synthetic construct
GGIGSDKLF

SEQ ID NO: 19022 - protein, 9 aa, synthetic construct
GGIGSDILN

SEQ ID NO: 19023 - protein, 9 aa, synthetic construct
GGIGSDILE

SEQ ID NO: 19024 - protein, 9 aa, synthetic construct
GGGGNDTMG

SEQ ID NO: 19025 - protein, 9 aa, synthetic construct
GGDGQDVFI

SEQ ID NO: 19026 - protein, 9 aa, synthetic construct
GGDGQDVFV

SEQ ID NO: 19027 - protein, 9 aa, synthetic construct
GGDGQDVII

SEQ ID NO: 19028 - protein, 9 aa, synthetic construct
GGIGSDRLA

SEQ ID NO: 19029 - protein, 9 aa, synthetic construct
GGIGSDRLR

SEQ ID NO: 19030 - protein, 9 aa, synthetic construct
GGIGSDRLS

SEQ ID NO: 19031 - protein, 9 aa, synthetic construct
GGDGQDSLL

SEQ ID NO: 19032 - protein, 9 aa, synthetic construct
GGDGQDSLD

SEQ ID NO: 19033 - protein, 9 aa, synthetic construct
GGIGSDTVQ

SEQ ID NO: 19034 - protein, 9 aa, synthetic construct
GGIGSDTMI

SEQ ID NO: 19035 - protein, 9 aa, synthetic construct
GGDGQDSLH

SEQ ID NO: 19036 - protein, 9 aa, synthetic construct
GGIGSDTLR

SEQ ID NO: 19037 - protein, 9 aa, synthetic construct
GGIGSDTLL

SEQ ID NO: 19038 - protein, 9 aa, synthetic construct
GGDGQDSLS

SEQ ID NO: 19039 - protein, 9 aa, synthetic construct
GGDGQDTIL

SEQ ID NO: 19040 - protein, 9 aa, synthetic construct
GGDGQDSLT

SEQ ID NO: 19041 - protein, 9 aa, synthetic construct
GGIGSDTAI

SEQ ID NO: 19042 - protein, 9 aa, synthetic construct
GGDGQDTIA

SEQ ID NO: 19043 - protein, 9 aa, synthetic construct
GGIGSDSLF

SEQ ID NO: 19044 - protein, 9 aa, synthetic construct
GGDGQDTIG

SEQ ID NO: 19045 - protein, 9 aa, synthetic construct
GGIGSDSIQ

SEQ ID NO: 19046 - protein, 9 aa, synthetic construct
GGIGDDHLT

SEQ ID NO: 19047 - protein, 9 aa, synthetic construct
GGIGDDFVY

SEQ ID NO: 19048 - protein, 9 aa, synthetic construct
GGIGDDFVK

SEQ ID NO: 19049 - protein, 9 aa, synthetic construct
GGGGWDTVT

SEQ ID NO: 19050 - protein, 9 aa, synthetic construct
GGGGWDRLT

SEQ ID NO: 19051 - protein, 9 aa, synthetic construct
GGGGWDRID

SEQ ID NO: 19052 - protein, 9 aa, synthetic construct
GGGGWDQLS

SEQ ID NO: 19053 - protein, 9 aa, synthetic construct
GGGGRDVMS

SEQ ID NO: 19054 - protein, 9 aa, synthetic construct
GGDGVDTLA

SEQ ID NO: 19055 - protein, 9 aa, synthetic construct
GGGGRDVVA

SEQ ID NO: 19056 - protein, 9 aa, synthetic construct
GGGGWDALY

SEQ ID NO: 19057 - protein, 9 aa, synthetic construct
GGGGVDYVE

SEQ ID NO: 19058 - protein, 9 aa, synthetic construct
GGDGVDTLH

SEQ ID NO: 19059 - protein, 9 aa, synthetic construct
GGGGVDYAT

SEQ ID NO: 19060 - protein, 9 aa, synthetic construct
GGGGVDVLR

SEQ ID NO: 19061 - protein, 9 aa, synthetic construct
GGGGVDVLN

SEQ ID NO: 19062 - protein, 9 aa, synthetic construct
GGGGVDVLF

SEQ ID NO: 19063 - protein, 9 aa, synthetic construct
GGGGVDVLD

SEQ ID NO: 19064 - protein, 9 aa, synthetic construct
GGEGADLIL

SEQ ID NO: 19065 - protein, 9 aa, synthetic construct
GGGGWDTLD

SEQ ID NO: 19066 - protein, 9 aa, synthetic construct
GGDGVDTIN

SEQ ID NO: 19067 - protein, 9 aa, synthetic construct
GGGGYDVLD

SEQ ID NO: 19068 - protein, 9 aa, synthetic construct
GGEGADLIR

SEQ ID NO: 19069 - protein, 9 aa, synthetic construct
GGDGVDRMV

SEQ ID NO: 19070 - protein, 9 aa, synthetic construct
GGDGVDRVI

SEQ ID NO: 19071 - protein, 9 aa, synthetic construct
GGGGYDTMA

SEQ ID NO: 19072 - protein, 9 aa, synthetic construct
GGDGVDSIF

SEQ ID NO: 19073 - protein, 9 aa, synthetic construct
GGDGVDSIV

SEQ ID NO: 19074 - protein, 9 aa, synthetic construct
GGGGYDTLI

SEQ ID NO: 19075 - protein, 9 aa, synthetic construct
GGGGYDRLY

SEQ ID NO: 19076 - protein, 9 aa, synthetic construct
GGGGRDVLR

SEQ ID NO: 19077 - protein, 9 aa, synthetic construct
GGDGVDSME

SEQ ID NO: 19078 - protein, 9 aa, synthetic construct
GGGGRDVLS

SEQ ID NO: 19079 - protein, 9 aa, synthetic construct
GGGGYDNLY

SEQ ID NO: 19080 - protein, 9 aa, synthetic construct
GGDGVDSVS

SEQ ID NO: 19081 - protein, 9 aa, synthetic construct
GGGGRDVLY

SEQ ID NO: 19082 - protein, 9 aa, synthetic construct
GGDGVDTAI

SEQ ID NO: 19083 - protein, 9 aa, synthetic construct
GGGGYDDLN

SEQ ID NO: 19084 - protein, 9 aa, synthetic construct
GGGGVDTYI

SEQ ID NO: 19085 - protein, 9 aa, synthetic construct
GGDGVDTLR

SEQ ID NO: 19086 - protein, 9 aa, synthetic construct
GGDGVDTMI

SEQ ID NO: 19087 - protein, 9 aa, synthetic construct
GGGGVDTMT

SEQ ID NO: 19088 - protein, 9 aa, synthetic construct
GGGGVDSLI

SEQ ID NO: 19089 - protein, 9 aa, synthetic construct
GGGGVDSIY

SEQ ID NO: 19090 - protein, 9 aa, synthetic construct
GGDGVDVLN

SEQ ID NO: 19091 - protein, 9 aa, synthetic construct
GGGGVDRLY

SEQ ID NO: 19092 - protein, 9 aa, synthetic construct
GGGGVDRLD

SEQ ID NO: 19093 - protein, 9 aa, synthetic construct
GGGGVDRIY

SEQ ID NO: 19094 - protein, 9 aa, synthetic construct
GGGGRDYID

SEQ ID NO: 19095 - protein, 9 aa, synthetic construct
GGDGVDVMT

SEQ ID NO: 19096 - protein, 9 aa, synthetic construct
GGGGVDQLY

SEQ ID NO: 19097 - protein, 9 aa, synthetic construct
GGDGVDWIK

SEQ ID NO: 19098 - protein, 9 aa, synthetic construct
GGGGVDQIS

SEQ ID NO: 19099 - protein, 9 aa, synthetic construct
GGGGVDNLH

SEQ ID NO: 19100 - protein, 9 aa, synthetic construct
GGDGVDWLY

SEQ ID NO: 19101 - protein, 9 aa, synthetic construct
GGEGADLFL

SEQ ID NO: 19102 - protein, 9 aa, synthetic construct
GGEGADLFG

SEQ ID NO: 19103 - protein, 9 aa, synthetic construct
GGGGVDSLY

SEQ ID NO: 19104 - protein, 9 aa, synthetic construct
GGDGVDVIL

SEQ ID NO: 19105 - protein, 9 aa, synthetic construct
GGGGVDTAD

SEQ ID NO: 19106 - protein, 9 aa, synthetic construct
GGGGVDTLH

SEQ ID NO: 19107 - protein, 9 aa, synthetic construct
GGDGVDTMS

SEQ ID NO: 19108 - protein, 9 aa, synthetic construct
GGGGVDTMI

SEQ ID NO: 19109 - protein, 9 aa, synthetic construct
GGGGVDTMA

SEQ ID NO: 19110 - protein, 9 aa, synthetic construct
GGEGADLIF

SEQ ID NO: 19111 - protein, 9 aa, synthetic construct
GGDGVDTVN

SEQ ID NO: 19112 - protein, 9 aa, synthetic construct
GGGGVDTLL

SEQ ID NO: 19113 - protein, 9 aa, synthetic construct
GGGGRDWIA

SEQ ID NO: 19114 - protein, 9 aa, synthetic construct
GGGGVDTAN

SEQ ID NO: 19115 - protein, 9 aa, synthetic construct
GGGGVDTIT

SEQ ID NO: 19116 - protein, 9 aa, synthetic construct
GGGGVDTID

SEQ ID NO: 19117 - protein, 9 aa, synthetic construct
GGGGRDWLH

SEQ ID NO: 19118 - protein, 9 aa, synthetic construct
GGGGRDWLS

SEQ ID NO: 19119 - protein, 9 aa, synthetic construct
GGGGVDTFI

SEQ ID NO: 19120 - protein, 9 aa, synthetic construct
GGGGVDTAV

SEQ ID NO: 19121 - protein, 9 aa, synthetic construct
GGDGVDRLV

SEQ ID NO: 19122 - protein, 9 aa, synthetic construct
GGGGRDVIY

SEQ ID NO: 19123 - protein, 9 aa, synthetic construct
GGDGVDYLS

SEQ ID NO: 19124 - protein, 9 aa, synthetic construct
GGHGDDLIG

SEQ ID NO: 19125 - protein, 9 aa, synthetic construct
GGHGDDKLY

SEQ ID NO: 19126 - protein, 9 aa, synthetic construct
GGEGADLMS

SEQ ID NO: 19127 - protein, 9 aa, synthetic construct
GGGGRDTIH

SEQ ID NO: 19128 - protein, 9 aa, synthetic construct
GGHGDDIYI

SEQ ID NO: 19129 - protein, 9 aa, synthetic construct
GGHGDDILV

SEQ ID NO: 19130 - protein, 9 aa, synthetic construct
GGHGDDILS

SEQ ID NO: 19131 - protein, 9 aa, synthetic construct
GGDGVDILR

SEQ ID NO: 19132 - protein, 9 aa, synthetic construct
GGGGRDTIR

SEQ ID NO: 19133 - protein, 9 aa, synthetic construct
GGGGRDTIV

SEQ ID NO: 19134 - protein, 9 aa, synthetic construct
GGHGDDGIT

SEQ ID NO: 19135 - protein, 9 aa, synthetic construct
GGDGVDIMN

SEQ ID NO: 19136 - protein, 9 aa, synthetic construct
GGHGDDEID

SEQ ID NO: 19137 - protein, 9 aa, synthetic construct
GGHGDDDLT

SEQ ID NO: 19138 - protein, 9 aa, synthetic construct
GGHGDDALY

SEQ ID NO: 19139 - protein, 9 aa, synthetic construct
GGDGVDKLI

SEQ ID NO: 19140 - protein, 9 aa, synthetic construct
GGHGDDLID

SEQ ID NO: 19141 - protein, 9 aa, synthetic construct
GGGGRDTID

SEQ ID NO: 19142 - protein, 9 aa, synthetic construct
GGDGVDRLN

SEQ ID NO: 19143 - protein, 9 aa, synthetic construct
GGHGDDLIQ

SEQ ID NO: 19144 - protein, 9 aa, synthetic construct
GGHGDDSLN

SEQ ID NO: 19145 - protein, 9 aa, synthetic construct
GGDGVDELW

SEQ ID NO: 19146 - protein, 9 aa, synthetic construct
GGGGRDSLI

SEQ ID NO: 19147 - protein, 9 aa, synthetic construct
GGDGVDFFI

SEQ ID NO: 19148 - protein, 9 aa, synthetic construct
GGHGDDRIN

SEQ ID NO: 19149 - protein, 9 aa, synthetic construct
GGDGVDFLV

SEQ ID NO: 19150 - protein, 9 aa, synthetic construct
GGGGRDTFA

SEQ ID NO: 19151 - protein, 9 aa, synthetic construct
GGGGRDTFI

SEQ ID NO: 19152 - protein, 9 aa, synthetic construct
GGGGRDTFL

SEQ ID NO: 19153 - protein, 9 aa, synthetic construct
GGHGDDLVV

SEQ ID NO: 19154 - protein, 9 aa, synthetic construct
GGHGDDLVI

SEQ ID NO: 19155 - protein, 9 aa, synthetic construct
GGHGDDLLT

SEQ ID NO: 19156 - protein, 9 aa, synthetic construct
GGHGDDLLR

SEQ ID NO: 19157 - protein, 9 aa, synthetic construct
GGHGDDLLE

SEQ ID NO: 19158 - protein, 9 aa, synthetic construct
GGHGDDLIT

SEQ ID NO: 19159 - protein, 9 aa, synthetic construct
GGGGRDTLF

SEQ ID NO: 19160 - protein, 9 aa, synthetic construct
GGHGADYFV

SEQ ID NO: 19161 - protein, 9 aa, synthetic construct
GGDGVDKLY

SEQ ID NO: 19162 - protein, 9 aa, synthetic construct
GGEGADLLV

SEQ ID NO: 19163 - protein, 9 aa, synthetic construct
GGDGVDNLK

SEQ ID NO: 19164 - protein, 9 aa, synthetic construct
GGHGADLMD

SEQ ID NO: 19165 - protein, 9 aa, synthetic construct
GGGGRDTYV

SEQ ID NO: 19166 - protein, 9 aa, synthetic construct
GGHGADLLL

SEQ ID NO: 19167 - protein, 9 aa, synthetic construct
GGGGRDVFE

SEQ ID NO: 19168 - protein, 9 aa, synthetic construct
GGDGVDQLR

SEQ ID NO: 19169 - protein, 9 aa, synthetic construct
GGGGRDVFI

SEQ ID NO: 19170 - protein, 9 aa, synthetic construct
GGHGADHLE

SEQ ID NO: 19171 - protein, 9 aa, synthetic construct
GGDGVDRLA

SEQ ID NO: 19172 - protein, 9 aa, synthetic construct
GGHGADGLD

SEQ ID NO: 19173 - protein, 9 aa, synthetic construct
GGHGADFLD

SEQ ID NO: 19174 - protein, 9 aa, synthetic construct
GGGGRDVIL

SEQ ID NO: 19175 - protein, 9 aa, synthetic construct
GGGGRDVIN

SEQ ID NO: 19176 - protein, 9 aa, synthetic construct
GGGGYDWLS

SEQ ID NO: 19177 - protein, 9 aa, synthetic construct
GGGGYDVLY

SEQ ID NO: 19178 - protein, 9 aa, synthetic construct
GGDGVDNLA

SEQ ID NO: 19179 - protein, 9 aa, synthetic construct
GGHGADRLA

SEQ ID NO: 19180 - protein, 9 aa, synthetic construct
GGHGADRLE

SEQ ID NO: 19181 - protein, 9 aa, synthetic construct
GGHGADTIH

SEQ ID NO: 19182 - protein, 9 aa, synthetic construct
GGHGADVID

SEQ ID NO: 19183 - protein, 9 aa, synthetic construct
GGDGVDLIA

SEQ ID NO: 19184 - protein, 9 aa, synthetic construct
GGDGVDLIH

SEQ ID NO: 19185 - protein, 9 aa, synthetic construct
GGHGADTMA

SEQ ID NO: 19186 - protein, 9 aa, synthetic construct
GGHGADTLK

SEQ ID NO: 19187 - protein, 9 aa, synthetic construct
GGDGVDLLN

SEQ ID NO: 19188 - protein, 9 aa, synthetic construct
GGHGADTID

SEQ ID NO: 19189 - protein, 9 aa, synthetic construct
GGHGADRLR

SEQ ID NO: 19190 - protein, 9 aa, synthetic construct
GGHGADTFV

SEQ ID NO: 19191 - protein, 9 aa, synthetic construct
GGHGADTFI

SEQ ID NO: 19192 - protein, 9 aa, synthetic construct
GGHGADSMD

SEQ ID NO: 19193 - protein, 9 aa, synthetic construct
GGGGRDTLV

SEQ ID NO: 19194 - protein, 9 aa, synthetic construct
GGDGVDMFV

SEQ ID NO: 19195 - protein, 9 aa, synthetic construct
GGHGADRME

SEQ ID NO: 19196 - protein, 9 aa, synthetic construct
GGDGVDYLD

SEQ ID NO: 19197 - protein, 9 aa, synthetic construct
GGGGVDLLT

SEQ ID NO: 19198 - protein, 9 aa, synthetic construct
GGGGQDTLY

SEQ ID NO: 19199 - protein, 9 aa, synthetic construct
GGGGSDVLA

SEQ ID NO: 19200 - protein, 9 aa, synthetic construct
GGGGSDVII

SEQ ID NO: 19201 - protein, 9 aa, synthetic construct
GGGGSDVFR

SEQ ID NO: 19202 - protein, 9 aa, synthetic construct
GGGGSDVFI

SEQ ID NO: 19203 - protein, 9 aa, synthetic construct
GGGGSDKIQ

SEQ ID NO: 19204 - protein, 9 aa, synthetic construct
GGGGSDTYL

SEQ ID NO: 19205 - protein, 9 aa, synthetic construct
GGGGSDTVL

SEQ ID NO: 19206 - protein, 9 aa, synthetic construct
GGEGADAMG

SEQ ID NO: 19207 - protein, 9 aa, synthetic construct
GGGGSDTVE

SEQ ID NO: 19208 - protein, 9 aa, synthetic construct
GGEGADCFV

SEQ ID NO: 19209 - protein, 9 aa, synthetic construct
GGGGSDTMV

SEQ ID NO: 19210 - protein, 9 aa, synthetic construct
GGGGSDKLI

SEQ ID NO: 19211 - protein, 9 aa, synthetic construct
GGGGSDKLR

SEQ ID NO: 19212 - protein, 9 aa, synthetic construct
GGGGSDTLA

SEQ ID NO: 19213 - protein, 9 aa, synthetic construct
GGGGSDTIG

SEQ ID NO: 19214 - protein, 9 aa, synthetic construct
GGEGADDLT

SEQ ID NO: 19215 - protein, 9 aa, synthetic construct
GGGGSDIYQ

SEQ ID NO: 19216 - protein, 9 aa, synthetic construct
GGGGSDVLF

SEQ ID NO: 19217 - protein, 9 aa, synthetic construct
GGEGADILI

SEQ ID NO: 19218 - protein, 9 aa, synthetic construct
GGGGSDILY

SEQ ID NO: 19219 - protein, 9 aa, synthetic construct
GGGGTDEAD

SEQ ID NO: 19220 - protein, 9 aa, synthetic construct
GGEGADILE

SEQ ID NO: 19221 - protein, 9 aa, synthetic construct
GGEGADIIS

SEQ ID NO: 19222 - protein, 9 aa, synthetic construct
GGEGADIIN

SEQ ID NO: 19223 - protein, 9 aa, synthetic construct
GGGGSDYLS

SEQ ID NO: 19224 - protein, 9 aa, synthetic construct
GGGGSDYLE

SEQ ID NO: 19225 - protein, 9 aa, synthetic construct
GGGGSDYID

SEQ ID NO: 19226 - protein, 9 aa, synthetic construct
GGGGSDYAL

SEQ ID NO: 19227 - protein, 9 aa, synthetic construct
GGGGSDWLI

SEQ ID NO: 19228 - protein, 9 aa, synthetic construct
GGGGSDILQ

SEQ ID NO: 19229 - protein, 9 aa, synthetic construct
GGGGSDWIE

SEQ ID NO: 19230 - protein, 9 aa, synthetic construct
GGDGYDYIE

SEQ ID NO: 19231 - protein, 9 aa, synthetic construct
GGGGSDVVS

SEQ ID NO: 19232 - protein, 9 aa, synthetic construct
GGEGADAFH

SEQ ID NO: 19233 - protein, 9 aa, synthetic construct
GGGGSDVMR

SEQ ID NO: 19234 - protein, 9 aa, synthetic construct
GGGGSDTFH

SEQ ID NO: 19235 - protein, 9 aa, synthetic construct
GGGGSDTFE

SEQ ID NO: 19236 - protein, 9 aa, synthetic construct
GGGGSDLID

SEQ ID NO: 19237 - protein, 9 aa, synthetic construct
GGGGSDTAV

SEQ ID NO: 19238 - protein, 9 aa, synthetic construct
GGGGSDRLF

SEQ ID NO: 19239 - protein, 9 aa, synthetic construct
GGEGADFLL

SEQ ID NO: 19240 - protein, 9 aa, synthetic construct
GGEGADFLQ

SEQ ID NO: 19241 - protein, 9 aa, synthetic construct
GGGGSDQLW

SEQ ID NO: 19242 - protein, 9 aa, synthetic construct
GGEGADHLY

SEQ ID NO: 19243 - protein, 9 aa, synthetic construct
GGEGADHLR

SEQ ID NO: 19244 - protein, 9 aa, synthetic construct
GGGGSDQLL

SEQ ID NO: 19245 - protein, 9 aa, synthetic construct
GGEGADHLI

SEQ ID NO: 19246 - protein, 9 aa, synthetic construct
GGEGADHLH

SEQ ID NO: 19247 - protein, 9 aa, synthetic construct
GGGGSDQLF

SEQ ID NO: 19248 - protein, 9 aa, synthetic construct
GGGGSDQFV

SEQ ID NO: 19249 - protein, 9 aa, synthetic construct
GGGGSDNLN

SEQ ID NO: 19250 - protein, 9 aa, synthetic construct
GGEGADHFD

SEQ ID NO: 19251 - protein, 9 aa, synthetic construct
GGGGSDMLD

SEQ ID NO: 19252 - protein, 9 aa, synthetic construct
GGEGADHIS

SEQ ID NO: 19253 - protein, 9 aa, synthetic construct
GGGGSDRLN

SEQ ID NO: 19254 - protein, 9 aa, synthetic construct
GGGGSDRLY

SEQ ID NO: 19255 - protein, 9 aa, synthetic construct
GGGGSDLLT

SEQ ID NO: 19256 - protein, 9 aa, synthetic construct
GGGGSDSLL

SEQ ID NO: 19257 - protein, 9 aa, synthetic construct
GGGGSDLIH

SEQ ID NO: 19258 - protein, 9 aa, synthetic construct
GGEGADEIH

SEQ ID NO: 19259 - protein, 9 aa, synthetic construct
GGEGADEII

SEQ ID NO: 19260 - protein, 9 aa, synthetic construct
GGGGSDSVI

SEQ ID NO: 19261 - protein, 9 aa, synthetic construct
GGEGADELF

SEQ ID NO: 19262 - protein, 9 aa, synthetic construct
GGGGSDSLR

SEQ ID NO: 19263 - protein, 9 aa, synthetic construct
GGGGSDSLH

SEQ ID NO: 19264 - protein, 9 aa, synthetic construct
GGEGADFIA

SEQ ID NO: 19265 - protein, 9 aa, synthetic construct
GGEGADELW

SEQ ID NO: 19266 - protein, 9 aa, synthetic construct
GGEGADELY

SEQ ID NO: 19267 - protein, 9 aa, synthetic construct
GGGGSDLIT

SEQ ID NO: 19268 - protein, 9 aa, synthetic construct
GGGGSDSIG

SEQ ID NO: 19269 - protein, 9 aa, synthetic construct
GGGGSDSIF

SEQ ID NO: 19270 - protein, 9 aa, synthetic construct
GGEGADEMW

SEQ ID NO: 19271 - protein, 9 aa, synthetic construct
GGGGTDEIC

SEQ ID NO: 19272 - protein, 9 aa, synthetic construct
GGGGSDIFV

SEQ ID NO: 19273 - protein, 9 aa, synthetic construct
GGGGVDLLI

SEQ ID NO: 19274 - protein, 9 aa, synthetic construct
GGGGTDVMT

SEQ ID NO: 19275 - protein, 9 aa, synthetic construct
GGGGSDEID

SEQ ID NO: 19276 - protein, 9 aa, synthetic construct
GGDGYDDFV

SEQ ID NO: 19277 - protein, 9 aa, synthetic construct
GGGGTDVLI

SEQ ID NO: 19278 - protein, 9 aa, synthetic construct
GGDGYDFIR

SEQ ID NO: 19279 - protein, 9 aa, synthetic construct
GGGGTDVFV

SEQ ID NO: 19280 - protein, 9 aa, synthetic construct
GGGGTDVFM

SEQ ID NO: 19281 - protein, 9 aa, synthetic construct
GGGGTDVAG

SEQ ID NO: 19282 - protein, 9 aa, synthetic construct
GGGGTDTVE

SEQ ID NO: 19283 - protein, 9 aa, synthetic construct
GGGGTDTLY

SEQ ID NO: 19284 - protein, 9 aa, synthetic construct
GGGGTDTLT

SEQ ID NO: 19285 - protein, 9 aa, synthetic construct
GGGGTDTLN

SEQ ID NO: 19286 - protein, 9 aa, synthetic construct
GGDGYDIAD

SEQ ID NO: 19287 - protein, 9 aa, synthetic construct
GGGGTDTIT

SEQ ID NO: 19288 - protein, 9 aa, synthetic construct
GGDGYDILN

SEQ ID NO: 19289 - protein, 9 aa, synthetic construct
GGDGYDIME

SEQ ID NO: 19290 - protein, 9 aa, synthetic construct
GGGGSDEFT

SEQ ID NO: 19291 - protein, 9 aa, synthetic construct
GGGGTDVVV

SEQ ID NO: 19292 - protein, 9 aa, synthetic construct
GGDGYDTLK

SEQ ID NO: 19293 - protein, 9 aa, synthetic construct
GGDGYDAIG

SEQ ID NO: 19294 - protein, 9 aa, synthetic construct
GGGGRDYLT

SEQ ID NO: 19295 - protein, 9 aa, synthetic construct
GGEGADKVS

SEQ ID NO: 19296 - protein, 9 aa, synthetic construct
GGDGWDFIQ

SEQ ID NO: 19297 - protein, 9 aa, synthetic construct
GGGGSDAIM

SEQ ID NO: 19298 - protein, 9 aa, synthetic construct
GGGGSDALH

SEQ ID NO: 19299 - protein, 9 aa, synthetic construct
GGDGWDMLA

SEQ ID NO: 19300 - protein, 9 aa, synthetic construct
GGGGSDALI

SEQ ID NO: 19301 - protein, 9 aa, synthetic construct
GGEGADKLT

SEQ ID NO: 19302 - protein, 9 aa, synthetic construct
GGDGWDTAT

SEQ ID NO: 19303 - protein, 9 aa, synthetic construct
GGDGWDTFI

SEQ ID NO: 19304 - protein, 9 aa, synthetic construct
GGDGWDTLM

SEQ ID NO: 19305 - protein, 9 aa, synthetic construct
GGGGTDYLY

SEQ ID NO: 19306 - protein, 9 aa, synthetic construct
GGEGADKFV

SEQ ID NO: 19307 - protein, 9 aa, synthetic construct
GGGGSDDMR

SEQ ID NO: 19308 - protein, 9 aa, synthetic construct
GGGGTDYAV

SEQ ID NO: 19309 - protein, 9 aa, synthetic construct
GGGGSDFAI

SEQ ID NO: 19310 - protein, 9 aa, synthetic construct
GGGGTDTAT

SEQ ID NO: 19311 - protein, 9 aa, synthetic construct
GGGGTDTAS

SEQ ID NO: 19312 - protein, 9 aa, synthetic construct
GGGGTDTAG

SEQ ID NO: 19313 - protein, 9 aa, synthetic construct
GGGGTDQLT

SEQ ID NO: 19314 - protein, 9 aa, synthetic construct
GGGGTDQLI

SEQ ID NO: 19315 - protein, 9 aa, synthetic construct
GGGGTDQLA

SEQ ID NO: 19316 - protein, 9 aa, synthetic construct
GGDGYDRID

SEQ ID NO: 19317 - protein, 9 aa, synthetic construct
GGGGTDNII

SEQ ID NO: 19318 - protein, 9 aa, synthetic construct
GGGGSDHLD

SEQ ID NO: 19319 - protein, 9 aa, synthetic construct
GGDGYDRLL

SEQ ID NO: 19320 - protein, 9 aa, synthetic construct
GGGGTDLLS

SEQ ID NO: 19321 - protein, 9 aa, synthetic construct
GGGGTDLLN

SEQ ID NO: 19322 - protein, 9 aa, synthetic construct
GGDGYDTAD

SEQ ID NO: 19323 - protein, 9 aa, synthetic construct
GGDGYDTFY

SEQ ID NO: 19324 - protein, 9 aa, synthetic construct
GGGGSDIFL

SEQ ID NO: 19325 - protein, 9 aa, synthetic construct
GGDGYDTIY

SEQ ID NO: 19326 - protein, 9 aa, synthetic construct
GGDGYDTLD

SEQ ID NO: 19327 - protein, 9 aa, synthetic construct
GGDGYDTLI

SEQ ID NO: 19328 - protein, 9 aa, synthetic construct
GGGGTDRFV

SEQ ID NO: 19329 - protein, 9 aa, synthetic construct
GGGGSDFLW

SEQ ID NO: 19330 - protein, 9 aa, synthetic construct
GGDGYDQIF

SEQ ID NO: 19331 - protein, 9 aa, synthetic construct
GGGGTDSLD

SEQ ID NO: 19332 - protein, 9 aa, synthetic construct
GGGGTDTAD

SEQ ID NO: 19333 - protein, 9 aa, synthetic construct
GGGGSDFLF

SEQ ID NO: 19334 - protein, 9 aa, synthetic construct
GGGGTDSLY

SEQ ID NO: 19335 - protein, 9 aa, synthetic construct
GGDGYDLLA

SEQ ID NO: 19336 - protein, 9 aa, synthetic construct
GGGGTDSLT

SEQ ID NO: 19337 - protein, 9 aa, synthetic construct
GGGGTDSLQ

SEQ ID NO: 19338 - protein, 9 aa, synthetic construct
GGGGTDSIL

SEQ ID NO: 19339 - protein, 9 aa, synthetic construct
GGGGTDRLF

SEQ ID NO: 19340 - protein, 9 aa, synthetic construct
GGDGYDLLR

SEQ ID NO: 19341 - protein, 9 aa, synthetic construct
GGGGTDRMR

SEQ ID NO: 19342 - protein, 9 aa, synthetic construct
GGGGTDRLT

SEQ ID NO: 19343 - protein, 9 aa, synthetic construct
GGGGSDFLQ

SEQ ID NO: 19344 - protein, 9 aa, synthetic construct
GGGGTDRLL

SEQ ID NO: 19345 - protein, 9 aa, synthetic construct
GGGGTDRLI

SEQ ID NO: 19346 - protein, 9 aa, synthetic construct
GGDGVDELR

SEQ ID NO: 19347 - protein, 9 aa, synthetic construct
GGHGDDTFL

SEQ ID NO: 19348 - protein, 9 aa, synthetic construct
GGGGRDSLE

SEQ ID NO: 19349 - protein, 9 aa, synthetic construct
GGIGADFMA

SEQ ID NO: 19350 - protein, 9 aa, synthetic construct
GGIGADFLS

SEQ ID NO: 19351 - protein, 9 aa, synthetic construct
GGIGADFFV

SEQ ID NO: 19352 - protein, 9 aa, synthetic construct
GGIGADELN

SEQ ID NO: 19353 - protein, 9 aa, synthetic construct
GGDGSDVLQ

SEQ ID NO: 19354 - protein, 9 aa, synthetic construct
GGIGADELI

SEQ ID NO: 19355 - protein, 9 aa, synthetic construct
GGDGSDVLS

SEQ ID NO: 19356 - protein, 9 aa, synthetic construct
GGIGADEFI

SEQ ID NO: 19357 - protein, 9 aa, synthetic construct
GGDGSDVLY

SEQ ID NO: 19358 - protein, 9 aa, synthetic construct
GGDGSDVMD

SEQ ID NO: 19359 - protein, 9 aa, synthetic construct
GGIGADDLD

SEQ ID NO: 19360 - protein, 9 aa, synthetic construct
GGGGRDELI

SEQ ID NO: 19361 - protein, 9 aa, synthetic construct
GGGGRDELT

SEQ ID NO: 19362 - protein, 9 aa, synthetic construct
GGDGSDVVY

SEQ ID NO: 19363 - protein, 9 aa, synthetic construct
GGIGADAFV

SEQ ID NO: 19364 - protein, 9 aa, synthetic construct
GGIGADAFI

SEQ ID NO: 19365 - protein, 9 aa, synthetic construct
GGIGADFLV

SEQ ID NO: 19366 - protein, 9 aa, synthetic construct
GGIGADHLT

SEQ ID NO: 19367 - protein, 9 aa, synthetic construct
GGGGRDDLS

SEQ ID NO: 19368 - protein, 9 aa, synthetic construct
GGDGSDVLE

SEQ ID NO: 19369 - protein, 9 aa, synthetic construct
GGGGRDDLW

SEQ ID NO: 19370 - protein, 9 aa, synthetic construct
GGDGSDVFV

SEQ ID NO: 19371 - protein, 9 aa, synthetic construct
GGDGSDVID

SEQ ID NO: 19372 - protein, 9 aa, synthetic construct
GGDGSDVIE

SEQ ID NO: 19373 - protein, 9 aa, synthetic construct
GGIGADKLY

SEQ ID NO: 19374 - protein, 9 aa, synthetic construct
GGDGSDVIL

SEQ ID NO: 19375 - protein, 9 aa, synthetic construct
GGIGADKLI

SEQ ID NO: 19376 - protein, 9 aa, synthetic construct
GGIGADKLF

SEQ ID NO: 19377 - protein, 9 aa, synthetic construct
GGEGADRIW

SEQ ID NO: 19378 - protein, 9 aa, synthetic construct
GGIGADIMI

SEQ ID NO: 19379 - protein, 9 aa, synthetic construct
GGIGADILV

SEQ ID NO: 19380 - protein, 9 aa, synthetic construct
GGIGADILN

SEQ ID NO: 19381 - protein, 9 aa, synthetic construct
GGDGSDVIT

SEQ ID NO: 19382 - protein, 9 aa, synthetic construct
GGDGSDVLA

SEQ ID NO: 19383 - protein, 9 aa, synthetic construct
GGIGADIIY

SEQ ID NO: 19384 - protein, 9 aa, synthetic construct
GGDGSDWAY

SEQ ID NO: 19385 - protein, 9 aa, synthetic construct
GGDGSDWIS

SEQ ID NO: 19386 - protein, 9 aa, synthetic construct
GGHGVDTLR

SEQ ID NO: 19387 - protein, 9 aa, synthetic construct
GGDGSDWLF

SEQ ID NO: 19388 - protein, 9 aa, synthetic construct
GGHGSDTIL

SEQ ID NO: 19389 - protein, 9 aa, synthetic construct
GGHGSDTIH

SEQ ID NO: 19390 - protein, 9 aa, synthetic construct
GGHGSDTIF

SEQ ID NO: 19391 - protein, 9 aa, synthetic construct
GGHGSDTFL

SEQ ID NO: 19392 - protein, 9 aa, synthetic construct
GGHGSDSLY

SEQ ID NO: 19393 - protein, 9 aa, synthetic construct
GGEGADQYW

SEQ ID NO: 19394 - protein, 9 aa, synthetic construct
GGHGSDLLD

SEQ ID NO: 19395 - protein, 9 aa, synthetic construct
GGDGTDALF

SEQ ID NO: 19396 - protein, 9 aa, synthetic construct
GGDGTDALY

SEQ ID NO: 19397 - protein, 9 aa, synthetic construct
GGHGRDVLN

SEQ ID NO: 19398 - protein, 9 aa, synthetic construct
GGHGRDVLA

SEQ ID NO: 19399 - protein, 9 aa, synthetic construct
GGDGTDELF

SEQ ID NO: 19400 - protein, 9 aa, synthetic construct
GGDGTDELV

SEQ ID NO: 19401 - protein, 9 aa, synthetic construct
GGGGRDILN

SEQ ID NO: 19402 - protein, 9 aa, synthetic construct
GGHGRDLLD

SEQ ID NO: 19403 - protein, 9 aa, synthetic construct
GGHGSDTLL

SEQ ID NO: 19404 - protein, 9 aa, synthetic construct
GGHGSDVLS

SEQ ID NO: 19405 - protein, 9 aa, synthetic construct
GGHGSDVLT

SEQ ID NO: 19406 - protein, 9 aa, synthetic construct
GGHGTDTLL

SEQ ID NO: 19407 - protein, 9 aa, synthetic construct
GGHGVDLLY

SEQ ID NO: 19408 - protein, 9 aa, synthetic construct
GGGGRDFIR

SEQ ID NO: 19409 - protein, 9 aa, synthetic construct
GGDGSDWLS

SEQ ID NO: 19410 - protein, 9 aa, synthetic construct
GGHGTDWLA

SEQ ID NO: 19411 - protein, 9 aa, synthetic construct
GGGGRDFLG

SEQ ID NO: 19412 - protein, 9 aa, synthetic construct
GGHGTDTLR

SEQ ID NO: 19413 - protein, 9 aa, synthetic construct
GGHGTDTII

SEQ ID NO: 19414 - protein, 9 aa, synthetic construct
GGDGSDYLS

SEQ ID NO: 19415 - protein, 9 aa, synthetic construct
GGDGSDYAD

SEQ ID NO: 19416 - protein, 9 aa, synthetic construct
GGHGTDTAD

SEQ ID NO: 19417 - protein, 9 aa, synthetic construct
GGDGSDYAL

SEQ ID NO: 19418 - protein, 9 aa, synthetic construct
GGDGSDYIW

SEQ ID NO: 19419 - protein, 9 aa, synthetic construct
GGHGSDYLR

SEQ ID NO: 19420 - protein, 9 aa, synthetic construct
GGEGADRIA

SEQ ID NO: 19421 - protein, 9 aa, synthetic construct
GGDGSDVAV

SEQ ID NO: 19422 - protein, 9 aa, synthetic construct
GGDGSDTYQ

SEQ ID NO: 19423 - protein, 9 aa, synthetic construct
GGHGDDTIT

SEQ ID NO: 19424 - protein, 9 aa, synthetic construct
GGDGSDSLV

SEQ ID NO: 19425 - protein, 9 aa, synthetic construct
GGGGQDVLY

SEQ ID NO: 19426 - protein, 9 aa, synthetic construct
GGGGQDVMF

SEQ ID NO: 19427 - protein, 9 aa, synthetic construct
GGIGADVLY

SEQ ID NO: 19428 - protein, 9 aa, synthetic construct
GGIGADVLT

SEQ ID NO: 19429 - protein, 9 aa, synthetic construct
GGIGADVLS

SEQ ID NO: 19430 - protein, 9 aa, synthetic construct
GGIGADVLE

SEQ ID NO: 19431 - protein, 9 aa, synthetic construct
GGGGQDYID

SEQ ID NO: 19432 - protein, 9 aa, synthetic construct
GGDGSDTAV

SEQ ID NO: 19433 - protein, 9 aa, synthetic construct
GGIGADVFR

SEQ ID NO: 19434 - protein, 9 aa, synthetic construct
GGGGQDYIH

SEQ ID NO: 19435 - protein, 9 aa, synthetic construct
GGIGADTVL

SEQ ID NO: 19436 - protein, 9 aa, synthetic construct
GGIGADTVD

SEQ ID NO: 19437 - protein, 9 aa, synthetic construct
GGIGADTMV

SEQ ID NO: 19438 - protein, 9 aa, synthetic construct
GGDGSDTFR

SEQ ID NO: 19439 - protein, 9 aa, synthetic construct
GGIGADTMK

SEQ ID NO: 19440 - protein, 9 aa, synthetic construct
GGIGADWME

SEQ ID NO: 19441 - protein, 9 aa, synthetic construct
GGIGADYMA

SEQ ID NO: 19442 - protein, 9 aa, synthetic construct
GGGGRDDIT

SEQ ID NO: 19443 - protein, 9 aa, synthetic construct
GGGGQDVLV

SEQ ID NO: 19444 - protein, 9 aa, synthetic construct
GGEGADRML

SEQ ID NO: 19445 - protein, 9 aa, synthetic construct
GGGGQDVFE

SEQ ID NO: 19446 - protein, 9 aa, synthetic construct
GGEGADRMA

SEQ ID NO: 19447 - protein, 9 aa, synthetic construct
GGGGQDVID

SEQ ID NO: 19448 - protein, 9 aa, synthetic construct
GGDGSDSFV

SEQ ID NO: 19449 - protein, 9 aa, synthetic construct
GGDGSDSID

SEQ ID NO: 19450 - protein, 9 aa, synthetic construct
GGDGSDSIG

SEQ ID NO: 19451 - protein, 9 aa, synthetic construct
GGDGSDSIL

SEQ ID NO: 19452 - protein, 9 aa, synthetic construct
GGGGQDVIY

SEQ ID NO: 19453 - protein, 9 aa, synthetic construct
GGIGDDDLT

SEQ ID NO: 19454 - protein, 9 aa, synthetic construct
GGDGSDSIV

SEQ ID NO: 19455 - protein, 9 aa, synthetic construct
GGIGDDDIY

SEQ ID NO: 19456 - protein, 9 aa, synthetic construct
GGIGDDALS

SEQ ID NO: 19457 - protein, 9 aa, synthetic construct
GGIGDDALL

SEQ ID NO: 19458 - protein, 9 aa, synthetic construct
GGIGDDAIF

SEQ ID NO: 19459 - protein, 9 aa, synthetic construct
GGDGSDTFS

SEQ ID NO: 19460 - protein, 9 aa, synthetic construct
GGDGSDTFT

SEQ ID NO: 19461 - protein, 9 aa, synthetic construct
GGIGADTLW

SEQ ID NO: 19462 - protein, 9 aa, synthetic construct
GGIGADTLR

SEQ ID NO: 19463 - protein, 9 aa, synthetic construct
GGDGSDTMV

SEQ ID NO: 19464 - protein, 9 aa, synthetic construct
GGIGADRLA

SEQ ID NO: 19465 - protein, 9 aa, synthetic construct
GGIGADRIN

SEQ ID NO: 19466 - protein, 9 aa, synthetic construct
GGIGADRFL

SEQ ID NO: 19467 - protein, 9 aa, synthetic construct
GGIGADRFD

SEQ ID NO: 19468 - protein, 9 aa, synthetic construct
GGIGADQMF

SEQ ID NO: 19469 - protein, 9 aa, synthetic construct
GGIGADQLS

SEQ ID NO: 19470 - protein, 9 aa, synthetic construct
GGGGRDALH

SEQ ID NO: 19471 - protein, 9 aa, synthetic construct
GGIGADQFS

SEQ ID NO: 19472 - protein, 9 aa, synthetic construct
GGIGADQFI

SEQ ID NO: 19473 - protein, 9 aa, synthetic construct
GGDGSDTVN

SEQ ID NO: 19474 - protein, 9 aa, synthetic construct
GGIGADPLT

SEQ ID NO: 19475 - protein, 9 aa, synthetic construct
GGIGADNLT

SEQ ID NO: 19476 - protein, 9 aa, synthetic construct
GGIGADNLQ

SEQ ID NO: 19477 - protein, 9 aa, synthetic construct
GGGGRDALS

SEQ ID NO: 19478 - protein, 9 aa, synthetic construct
GGDGSDTMT

SEQ ID NO: 19479 - protein, 9 aa, synthetic construct
GGDGSDTMQ

SEQ ID NO: 19480 - protein, 9 aa, synthetic construct
GGDGSDTML

SEQ ID NO: 19481 - protein, 9 aa, synthetic construct
GGIGADTFI

SEQ ID NO: 19482 - protein, 9 aa, synthetic construct
GGDGSDTFV

SEQ ID NO: 19483 - protein, 9 aa, synthetic construct
GGDGSDTIH

SEQ ID NO: 19484 - protein, 9 aa, synthetic construct
GGDGSDTIK

SEQ ID NO: 19485 - protein, 9 aa, synthetic construct
GGIGADTIG

SEQ ID NO: 19486 - protein, 9 aa, synthetic construct
GGIGADTID

SEQ ID NO: 19487 - protein, 9 aa, synthetic construct
GGIGADTIA

SEQ ID NO: 19488 - protein, 9 aa, synthetic construct
GGGGQDYLD

SEQ ID NO: 19489 - protein, 9 aa, synthetic construct
GGIGADSFI

SEQ ID NO: 19490 - protein, 9 aa, synthetic construct
GGGGQDYLF

SEQ ID NO: 19491 - protein, 9 aa, synthetic construct
GGIGADSVS

SEQ ID NO: 19492 - protein, 9 aa, synthetic construct
GGDGSDTLK

SEQ ID NO: 19493 - protein, 9 aa, synthetic construct
GGIGADSLL

SEQ ID NO: 19494 - protein, 9 aa, synthetic construct
GGIGADSLH

SEQ ID NO: 19495 - protein, 9 aa, synthetic construct
GGDGSDTLQ

SEQ ID NO: 19496 - protein, 9 aa, synthetic construct
GGHGRDHLI

SEQ ID NO: 19497 - protein, 9 aa, synthetic construct
GGHGRDHFV

SEQ ID NO: 19498 - protein, 9 aa, synthetic construct
GGHGQDVLG

SEQ ID NO: 19499 - protein, 9 aa, synthetic construct
GGDGTDTLR

SEQ ID NO: 19500 - protein, 9 aa, synthetic construct
GGHGHDTLI

SEQ ID NO: 19501 - protein, 9 aa, synthetic construct
GGDGTDTVL

SEQ ID NO: 19502 - protein, 9 aa, synthetic construct
GGHGHDRLS

SEQ ID NO: 19503 - protein, 9 aa, synthetic construct
GGGGRDRIA

SEQ ID NO: 19504 - protein, 9 aa, synthetic construct
GGHGGDWLF

SEQ ID NO: 19505 - protein, 9 aa, synthetic construct
GGGGRDRIF

SEQ ID NO: 19506 - protein, 9 aa, synthetic construct
GGDGTDVFV

SEQ ID NO: 19507 - protein, 9 aa, synthetic construct
GGDGTDVII

SEQ ID NO: 19508 - protein, 9 aa, synthetic construct
GGDGTDVLD

SEQ ID NO: 19509 - protein, 9 aa, synthetic construct
GGHGFDTLY

SEQ ID NO: 19510 - protein, 9 aa, synthetic construct
GGDGTDVLI

SEQ ID NO: 19511 - protein, 9 aa, synthetic construct
GGDGTDVLL

SEQ ID NO: 19512 - protein, 9 aa, synthetic construct
GGHGEDWLE

SEQ ID NO: 19513 - protein, 9 aa, synthetic construct
GGDGTDVLV

SEQ ID NO: 19514 - protein, 9 aa, synthetic construct
GGHGEDVLK

SEQ ID NO: 19515 - protein, 9 aa, synthetic construct
GGHGHDTLL

SEQ ID NO: 19516 - protein, 9 aa, synthetic construct
GGHGHDVID

SEQ ID NO: 19517 - protein, 9 aa, synthetic construct
GGGGRDKIN

SEQ ID NO: 19518 - protein, 9 aa, synthetic construct
GGHGHDVLA

SEQ ID NO: 19519 - protein, 9 aa, synthetic construct
GGDGTDTAE

SEQ ID NO: 19520 - protein, 9 aa, synthetic construct
GGGGRDQIL

SEQ ID NO: 19521 - protein, 9 aa, synthetic construct
GGEGADNIK

SEQ ID NO: 19522 - protein, 9 aa, synthetic construct
GGHGLDVVA

SEQ ID NO: 19523 - protein, 9 aa, synthetic construct
GGHGLDTLY

SEQ ID NO: 19524 - protein, 9 aa, synthetic construct
GGGGRDQLD

SEQ ID NO: 19525 - protein, 9 aa, synthetic construct
GGHGKDVLI

SEQ ID NO: 19526 - protein, 9 aa, synthetic construct
GGGGRDQLL

SEQ ID NO: 19527 - protein, 9 aa, synthetic construct
GGDGTDTIF

SEQ ID NO: 19528 - protein, 9 aa, synthetic construct
GGDGTDTIL

SEQ ID NO: 19529 - protein, 9 aa, synthetic construct
GGHGKDRLV

SEQ ID NO: 19530 - protein, 9 aa, synthetic construct
GGHGKDRLH

SEQ ID NO: 19531 - protein, 9 aa, synthetic construct
GGEGADMLT

SEQ ID NO: 19532 - protein, 9 aa, synthetic construct
GGDGTDTLG

SEQ ID NO: 19533 - protein, 9 aa, synthetic construct
GGHGHDVLS

SEQ ID NO: 19534 - protein, 9 aa, synthetic construct
GGHGEDTLT

SEQ ID NO: 19535 - protein, 9 aa, synthetic construct
GGHGEDTAV

SEQ ID NO: 19536 - protein, 9 aa, synthetic construct
GGHGEDRLI

SEQ ID NO: 19537 - protein, 9 aa, synthetic construct
GGHGEDLLV

SEQ ID NO: 19538 - protein, 9 aa, synthetic construct
GGHGDDTYD

SEQ ID NO: 19539 - protein, 9 aa, synthetic construct
GGHGDDTVT

SEQ ID NO: 19540 - protein, 9 aa, synthetic construct
GGGGRDSFV

SEQ ID NO: 19541 - protein, 9 aa, synthetic construct
GGGGRDSIA

SEQ ID NO: 19542 - protein, 9 aa, synthetic construct
GGHGDDTMI

SEQ ID NO: 19543 - protein, 9 aa, synthetic construct
GGHGDDTLV

SEQ ID NO: 19544 - protein, 9 aa, synthetic construct
GGDGVDCLD

SEQ ID NO: 19545 - protein, 9 aa, synthetic construct
GGHGDDTLR

SEQ ID NO: 19546 - protein, 9 aa, synthetic construct
GGHGDDTLN

SEQ ID NO: 19547 - protein, 9 aa, synthetic construct
GGGGRDSIT

SEQ ID NO: 19548 - protein, 9 aa, synthetic construct
GGDGVDDLA

SEQ ID NO: 19549 - protein, 9 aa, synthetic construct
GGDGVDDLQ

SEQ ID NO: 19550 - protein, 9 aa, synthetic construct
GGGGRDSLA

SEQ ID NO: 19551 - protein, 9 aa, synthetic construct
GGHGDDTLA

SEQ ID NO: 19552 - protein, 9 aa, synthetic construct
GGHGDDTIV

SEQ ID NO: 19553 - protein, 9 aa, synthetic construct
GGDGVDALY

SEQ ID NO: 19554 - protein, 9 aa, synthetic construct
GGHGDDVIN

SEQ ID NO: 19555 - protein, 9 aa, synthetic construct
GGHGDDVLF

SEQ ID NO: 19556 - protein, 9 aa, synthetic construct
GGHGDDYLE

SEQ ID NO: 19557 - protein, 9 aa, synthetic construct
GGHGEDLLA

SEQ ID NO: 19558 - protein, 9 aa, synthetic construct
GGGGRDRLK

SEQ ID NO: 19559 - protein, 9 aa, synthetic construct
GGHGEDEIH

SEQ ID NO: 19560 - protein, 9 aa, synthetic construct
GGGGRDRLL

SEQ ID NO: 19561 - protein, 9 aa, synthetic construct
GGEGADLYI

SEQ ID NO: 19562 - protein, 9 aa, synthetic construct
GGDGTDYLS

SEQ ID NO: 19563 - protein, 9 aa, synthetic construct
GGHGDDWLS

SEQ ID NO: 19564 - protein, 9 aa, synthetic construct
GGHGDDVLH

SEQ ID NO: 19565 - protein, 9 aa, synthetic construct
GGGGRDRLS

SEQ ID NO: 19566 - protein, 9 aa, synthetic construct
GGHGDDVVL

SEQ ID NO: 19567 - protein, 9 aa, synthetic construct
GGHGDDVLR

SEQ ID NO: 19568 - protein, 9 aa, synthetic construct
GGHGDDVLQ

SEQ ID NO: 19569 - protein, 9 aa, synthetic construct
GGHGDDVLL

SEQ ID NO: 19570 - protein, 9 aa, synthetic construct
GGGGRDRML

SEQ ID NO: 19571 - protein, 9 aa, synthetic construct
GGHGNDELA

SEQ ID NO: 19572 - protein, 9 aa, synthetic construct
GGHGNDELH

SEQ ID NO: 19573 - protein, 9 aa, synthetic construct
GGDGTDTAA

SEQ ID NO: 19574 - protein, 9 aa, synthetic construct
GGHGNDSLS

SEQ ID NO: 19575 - protein, 9 aa, synthetic construct
GGHGNDVIG

SEQ ID NO: 19576 - protein, 9 aa, synthetic construct
GGHGNDVIE

SEQ ID NO: 19577 - protein, 9 aa, synthetic construct
GGGGRDLIH

SEQ ID NO: 19578 - protein, 9 aa, synthetic construct
GGGGRDLII

SEQ ID NO: 19579 - protein, 9 aa, synthetic construct
GGEGADQLA

SEQ ID NO: 19580 - protein, 9 aa, synthetic construct
GGHGNDVFR

SEQ ID NO: 19581 - protein, 9 aa, synthetic construct
GGGGRDLIL

SEQ ID NO: 19582 - protein, 9 aa, synthetic construct
GGHGNDTVN

SEQ ID NO: 19583 - protein, 9 aa, synthetic construct
GGHGNDTVI

SEQ ID NO: 19584 - protein, 9 aa, synthetic construct
GGGGRDLIV

SEQ ID NO: 19585 - protein, 9 aa, synthetic construct
GGHGNDTLV

SEQ ID NO: 19586 - protein, 9 aa, synthetic construct
GGHGNDTLT

SEQ ID NO: 19587 - protein, 9 aa, synthetic construct
GGGGRDLIY

SEQ ID NO: 19588 - protein, 9 aa, synthetic construct
GGHGNDTIN

SEQ ID NO: 19589 - protein, 9 aa, synthetic construct
GGDGTDLLL

SEQ ID NO: 19590 - protein, 9 aa, synthetic construct
GGEGADQLD

SEQ ID NO: 19591 - protein, 9 aa, synthetic construct
GGDGTDKIK

SEQ ID NO: 19592 - protein, 9 aa, synthetic construct
GGHGNDVLH

SEQ ID NO: 19593 - protein, 9 aa, synthetic construct
GGDGTDILQ

SEQ ID NO: 19594 - protein, 9 aa, synthetic construct
GGDGTDHLY

SEQ ID NO: 19595 - protein, 9 aa, synthetic construct
GGDGTDIAS

SEQ ID NO: 19596 - protein, 9 aa, synthetic construct
GGGGRDKLT

SEQ ID NO: 19597 - protein, 9 aa, synthetic construct
GGEGADQLL

SEQ ID NO: 19598 - protein, 9 aa, synthetic construct
GGHGPDILT

SEQ ID NO: 19599 - protein, 9 aa, synthetic construct
GGHGNDYLY

SEQ ID NO: 19600 - protein, 9 aa, synthetic construct
GGHGNDYLI

SEQ ID NO: 19601 - protein, 9 aa, synthetic construct
GGHGNDVLW

SEQ ID NO: 19602 - protein, 9 aa, synthetic construct
GGGGRDKLW

SEQ ID NO: 19603 - protein, 9 aa, synthetic construct
GGGGRDKLY

SEQ ID NO: 19604 - protein, 9 aa, synthetic construct
GGHGNDWLD

SEQ ID NO: 19605 - protein, 9 aa, synthetic construct
GGDGTDILW

SEQ ID NO: 19606 - protein, 9 aa, synthetic construct
GGHGNDVMR

SEQ ID NO: 19607 - protein, 9 aa, synthetic construct
GGGGRDKVL

SEQ ID NO: 19608 - protein, 9 aa, synthetic construct
GGGGRDLLF

SEQ ID NO: 19609 - protein, 9 aa, synthetic construct
GGGGRDLLH

SEQ ID NO: 19610 - protein, 9 aa, synthetic construct
GGDGTDSVT

SEQ ID NO: 19611 - protein, 9 aa, synthetic construct
GGDGTDLMY

SEQ ID NO: 19612 - protein, 9 aa, synthetic construct
GGHGNDLFI

SEQ ID NO: 19613 - protein, 9 aa, synthetic construct
GGHGNDKLW

SEQ ID NO: 19614 - protein, 9 aa, synthetic construct
GGHGNDKLV

SEQ ID NO: 19615 - protein, 9 aa, synthetic construct
GGHGNDIYV

SEQ ID NO: 19616 - protein, 9 aa, synthetic construct
GGHGNDIMN

SEQ ID NO: 19617 - protein, 9 aa, synthetic construct
GGHGNDILI

SEQ ID NO: 19618 - protein, 9 aa, synthetic construct
GGGGRDNLN

SEQ ID NO: 19619 - protein, 9 aa, synthetic construct
GGHGNDIID

SEQ ID NO: 19620 - protein, 9 aa, synthetic construct
GGEGADNLA

SEQ ID NO: 19621 - protein, 9 aa, synthetic construct
GGDGTDSIE

SEQ ID NO: 19622 - protein, 9 aa, synthetic construct
GGHGNDHLD

SEQ ID NO: 19623 - protein, 9 aa, synthetic construct
GGHGNDGLF

SEQ ID NO: 19624 - protein, 9 aa, synthetic construct
GGDGTDSLT

SEQ ID NO: 19625 - protein, 9 aa, synthetic construct
GGHGNDFLK

SEQ ID NO: 19626 - protein, 9 aa, synthetic construct
GGGGRDQID

SEQ ID NO: 19627 - protein, 9 aa, synthetic construct
GGDGTDRLI

SEQ ID NO: 19628 - protein, 9 aa, synthetic construct
GGHGNDLLH

SEQ ID NO: 19629 - protein, 9 aa, synthetic construct
GGHGNDLLL

SEQ ID NO: 19630 - protein, 9 aa, synthetic construct
GGHGNDQMD

SEQ ID NO: 19631 - protein, 9 aa, synthetic construct
GGGGRDLLM

SEQ ID NO: 19632 - protein, 9 aa, synthetic construct
GGDGTDMLD

SEQ ID NO: 19633 - protein, 9 aa, synthetic construct
GGHGNDRME

SEQ ID NO: 19634 - protein, 9 aa, synthetic construct
GGHGNDRLV

SEQ ID NO: 19635 - protein, 9 aa, synthetic construct
GGHGNDRLL

SEQ ID NO: 19636 - protein, 9 aa, synthetic construct
GGHGNDRIY

SEQ ID NO: 19637 - protein, 9 aa, synthetic construct
GGEGADQFN

SEQ ID NO: 19638 - protein, 9 aa, synthetic construct
GGGGRDNLF

SEQ ID NO: 19639 - protein, 9 aa, synthetic construct
GGEGADQFI

SEQ ID NO: 19640 - protein, 9 aa, synthetic construct
GGDGTDQAS

SEQ ID NO: 19641 - protein, 9 aa, synthetic construct
GGDGTDQLF

SEQ ID NO: 19642 - protein, 9 aa, synthetic construct
GGGGRDMLS

SEQ ID NO: 19643 - protein, 9 aa, synthetic construct
GGDGTDRIF

SEQ ID NO: 19644 - protein, 9 aa, synthetic construct
GGDGTDRLE

SEQ ID NO: 19645 - protein, 9 aa, synthetic construct
GGDGNDWIV

SEQ ID NO: 19646 - protein, 9 aa, synthetic construct
GGDGNDWIQ

SEQ ID NO: 19647 - protein, 9 aa, synthetic construct
GGDGHDFFY

SEQ ID NO: 19648 - protein, 9 aa, synthetic construct
GGLGGDIIK

SEQ ID NO: 19649 - protein, 9 aa, synthetic construct
GGLGGDELA

SEQ ID NO: 19650 - protein, 9 aa, synthetic construct
GGLGGDEFV

SEQ ID NO: 19651 - protein, 9 aa, synthetic construct
GGDGKDRLL

SEQ ID NO: 19652 - protein, 9 aa, synthetic construct
GGDGKDRLN

SEQ ID NO: 19653 - protein, 9 aa, synthetic construct
GGDGKDRLT

SEQ ID NO: 19654 - protein, 9 aa, synthetic construct
GGLGGDALT

SEQ ID NO: 19655 - protein, 9 aa, synthetic construct
GGDGKDRLV

SEQ ID NO: 19656 - protein, 9 aa, synthetic construct
GGDGKDSID

SEQ ID NO: 19657 - protein, 9 aa, synthetic construct
GGLGGDAFV

SEQ ID NO: 19658 - protein, 9 aa, synthetic construct
GGLGGDAFI

SEQ ID NO: 19659 - protein, 9 aa, synthetic construct
GGDGKDSIL

SEQ ID NO: 19660 - protein, 9 aa, synthetic construct
GGLGFDVVS

SEQ ID NO: 19661 - protein, 9 aa, synthetic construct
GGGGNDAIV

SEQ ID NO: 19662 - protein, 9 aa, synthetic construct
GGDGKDSLD

SEQ ID NO: 19663 - protein, 9 aa, synthetic construct
GGDGKDSLH

SEQ ID NO: 19664 - protein, 9 aa, synthetic construct
GGGGNDAII

SEQ ID NO: 19665 - protein, 9 aa, synthetic construct
GGDGKDRFV

SEQ ID NO: 19666 - protein, 9 aa, synthetic construct
GGLGGDRLY

SEQ ID NO: 19667 - protein, 9 aa, synthetic construct
GGLGGDILR

SEQ ID NO: 19668 - protein, 9 aa, synthetic construct
GGLGGDRLS

SEQ ID NO: 19669 - protein, 9 aa, synthetic construct
GGDGKDNFY

SEQ ID NO: 19670 - protein, 9 aa, synthetic construct
GGLGGDQLR

SEQ ID NO: 19671 - protein, 9 aa, synthetic construct
GGLGGDQIW

SEQ ID NO: 19672 - protein, 9 aa, synthetic construct
GGEGDDFIG

SEQ ID NO: 19673 - protein, 9 aa, synthetic construct
GGLGGDLLW

SEQ ID NO: 19674 - protein, 9 aa, synthetic construct
GGEGDDFIF

SEQ ID NO: 19675 - protein, 9 aa, synthetic construct
GGLGGDLLN

SEQ ID NO: 19676 - protein, 9 aa, synthetic construct
GGLGGDLLL

SEQ ID NO: 19677 - protein, 9 aa, synthetic construct
GGDGKDQLF

SEQ ID NO: 19678 - protein, 9 aa, synthetic construct
GGDGKDQLN

SEQ ID NO: 19679 - protein, 9 aa, synthetic construct
GGGGMDYME

SEQ ID NO: 19680 - protein, 9 aa, synthetic construct
GGLGGDIMR

SEQ ID NO: 19681 - protein, 9 aa, synthetic construct
GGDGKDQLW

SEQ ID NO: 19682 - protein, 9 aa, synthetic construct
GGDGKDQLY

SEQ ID NO: 19683 - protein, 9 aa, synthetic construct
GGDGKDSLQ

SEQ ID NO: 19684 - protein, 9 aa, synthetic construct
GGDGKDSVD

SEQ ID NO: 19685 - protein, 9 aa, synthetic construct
GGDGKDSVL

SEQ ID NO: 19686 - protein, 9 aa, synthetic construct
GGLGFDTVS

SEQ ID NO: 19687 - protein, 9 aa, synthetic construct
GGLGEDVMF

SEQ ID NO: 19688 - protein, 9 aa, synthetic construct
GGLGEDVLN

SEQ ID NO: 19689 - protein, 9 aa, synthetic construct
GGLGEDVLI

SEQ ID NO: 19690 - protein, 9 aa, synthetic construct
GGLGEDVLE

SEQ ID NO: 19691 - protein, 9 aa, synthetic construct
GGLGEDVLD

SEQ ID NO: 19692 - protein, 9 aa, synthetic construct
GGDGKDVIF

SEQ ID NO: 19693 - protein, 9 aa, synthetic construct
GGEGDDEVF

SEQ ID NO: 19694 - protein, 9 aa, synthetic construct
GGLGEDVAV

SEQ ID NO: 19695 - protein, 9 aa, synthetic construct
GGGGNDAVL

SEQ ID NO: 19696 - protein, 9 aa, synthetic construct
GGLGEDTLS

SEQ ID NO: 19697 - protein, 9 aa, synthetic construct
GGLGEDTLQ

SEQ ID NO: 19698 - protein, 9 aa, synthetic construct
GGEGDDEME

SEQ ID NO: 19699 - protein, 9 aa, synthetic construct
GGLGEDTLE

SEQ ID NO: 19700 - protein, 9 aa, synthetic construct
GGDGKDVLR

SEQ ID NO: 19701 - protein, 9 aa, synthetic construct
GGDGKDVLT

SEQ ID NO: 19702 - protein, 9 aa, synthetic construct
GGLGEDVML

SEQ ID NO: 19703 - protein, 9 aa, synthetic construct
GGDGKDVFF

SEQ ID NO: 19704 - protein, 9 aa, synthetic construct
GGDGKDVFA

SEQ ID NO: 19705 - protein, 9 aa, synthetic construct
GGLGFDSAI

SEQ ID NO: 19706 - protein, 9 aa, synthetic construct
GGLGFDTMT

SEQ ID NO: 19707 - protein, 9 aa, synthetic construct
GGLGFDTLT

SEQ ID NO: 19708 - protein, 9 aa, synthetic construct
GGLGFDTLN

SEQ ID NO: 19709 - protein, 9 aa, synthetic construct
GGGGNDALH

SEQ ID NO: 19710 - protein, 9 aa, synthetic construct
GGDGKDTID

SEQ ID NO: 19711 - protein, 9 aa, synthetic construct
GGDGKDTII

SEQ ID NO: 19712 - protein, 9 aa, synthetic construct
GGDGKDTIY

SEQ ID NO: 19713 - protein, 9 aa, synthetic construct
GGLGFDALT

SEQ ID NO: 19714 - protein, 9 aa, synthetic construct
GGLGFDRLD

SEQ ID NO: 19715 - protein, 9 aa, synthetic construct
GGGGNDALR

SEQ ID NO: 19716 - protein, 9 aa, synthetic construct
GGLGFDLLV

SEQ ID NO: 19717 - protein, 9 aa, synthetic construct
GGLGFDKLS

SEQ ID NO: 19718 - protein, 9 aa, synthetic construct
GGDGKDTLQ

SEQ ID NO: 19719 - protein, 9 aa, synthetic construct
GGDGKDTLR

SEQ ID NO: 19720 - protein, 9 aa, synthetic construct
GGLGGDRLT

SEQ ID NO: 19721 - protein, 9 aa, synthetic construct
GGDGKDMLY

SEQ ID NO: 19722 - protein, 9 aa, synthetic construct
GGDGKDVLW

SEQ ID NO: 19723 - protein, 9 aa, synthetic construct
GGLGHDRMV

SEQ ID NO: 19724 - protein, 9 aa, synthetic construct
GGLGHDRLE

SEQ ID NO: 19725 - protein, 9 aa, synthetic construct
GGDGKDDVN

SEQ ID NO: 19726 - protein, 9 aa, synthetic construct
GGLGHDQLR

SEQ ID NO: 19727 - protein, 9 aa, synthetic construct
GGLGHDQLF

SEQ ID NO: 19728 - protein, 9 aa, synthetic construct
GGLGHDMLL

SEQ ID NO: 19729 - protein, 9 aa, synthetic construct
GGLGHDMIR

SEQ ID NO: 19730 - protein, 9 aa, synthetic construct
GGEGDDFVK

SEQ ID NO: 19731 - protein, 9 aa, synthetic construct
GGLGHDLLR

SEQ ID NO: 19732 - protein, 9 aa, synthetic construct
GGLGHDLLN

SEQ ID NO: 19733 - protein, 9 aa, synthetic construct
GGGGLDTLV

SEQ ID NO: 19734 - protein, 9 aa, synthetic construct
GGGGLDTLY

SEQ ID NO: 19735 - protein, 9 aa, synthetic construct
GGLGHDKFI

SEQ ID NO: 19736 - protein, 9 aa, synthetic construct
GGDGKDFMV

SEQ ID NO: 19737 - protein, 9 aa, synthetic construct
GGGGLDTYR

SEQ ID NO: 19738 - protein, 9 aa, synthetic construct
GGDGKDIFS

SEQ ID NO: 19739 - protein, 9 aa, synthetic construct
GGLGHDRLN

SEQ ID NO: 19740 - protein, 9 aa, synthetic construct
GGLGHDRVF

SEQ ID NO: 19741 - protein, 9 aa, synthetic construct
GGLGGDRMT

SEQ ID NO: 19742 - protein, 9 aa, synthetic construct
GGLGHDRYV

SEQ ID NO: 19743 - protein, 9 aa, synthetic construct
GGLGIDALT

SEQ ID NO: 19744 - protein, 9 aa, synthetic construct
GGEGDDHIR

SEQ ID NO: 19745 - protein, 9 aa, synthetic construct
GGEGDDHID

SEQ ID NO: 19746 - protein, 9 aa, synthetic construct
GGLGHDVMR

SEQ ID NO: 19747 - protein, 9 aa, synthetic construct
GGLGHDVLY

SEQ ID NO: 19748 - protein, 9 aa, synthetic construct
GGLGHDVLS

SEQ ID NO: 19749 - protein, 9 aa, synthetic construct
GGGGLDRVA

SEQ ID NO: 19750 - protein, 9 aa, synthetic construct
GGDGIDWIQ

SEQ ID NO: 19751 - protein, 9 aa, synthetic construct
GGEGDDGLD

SEQ ID NO: 19752 - protein, 9 aa, synthetic construct
GGLGHDTLF

SEQ ID NO: 19753 - protein, 9 aa, synthetic construct
GGGGLDTIY

SEQ ID NO: 19754 - protein, 9 aa, synthetic construct
GGLGHDTIN

SEQ ID NO: 19755 - protein, 9 aa, synthetic construct
GGEGDDGFF

SEQ ID NO: 19756 - protein, 9 aa, synthetic construct
GGDGIDYLY

SEQ ID NO: 19757 - protein, 9 aa, synthetic construct
GGEGDDFYE

SEQ ID NO: 19758 - protein, 9 aa, synthetic construct
GGDGKDIID

SEQ ID NO: 19759 - protein, 9 aa, synthetic construct
GGEGDDFMD

SEQ ID NO: 19760 - protein, 9 aa, synthetic construct
GGGGLDVLN

SEQ ID NO: 19761 - protein, 9 aa, synthetic construct
GGDGKDILD

SEQ ID NO: 19762 - protein, 9 aa, synthetic construct
GGDGKDLLE

SEQ ID NO: 19763 - protein, 9 aa, synthetic construct
GGLGGDTLK

SEQ ID NO: 19764 - protein, 9 aa, synthetic construct
GGLGGDTLI

SEQ ID NO: 19765 - protein, 9 aa, synthetic construct
GGGGMDLVS

SEQ ID NO: 19766 - protein, 9 aa, synthetic construct
GGLGGDTLE

SEQ ID NO: 19767 - protein, 9 aa, synthetic construct
GGGGMDRLL

SEQ ID NO: 19768 - protein, 9 aa, synthetic construct
GGLGGDTIN

SEQ ID NO: 19769 - protein, 9 aa, synthetic construct
GGDGKDLLL

SEQ ID NO: 19770 - protein, 9 aa, synthetic construct
GGLGGDTIE

SEQ ID NO: 19771 - protein, 9 aa, synthetic construct
GGDGKDLLS

SEQ ID NO: 19772 - protein, 9 aa, synthetic construct
GGLGGDSLY

SEQ ID NO: 19773 - protein, 9 aa, synthetic construct
GGGGMDTLF

SEQ ID NO: 19774 - protein, 9 aa, synthetic construct
GGLGGDSLF

SEQ ID NO: 19775 - protein, 9 aa, synthetic construct
GGLGGDSLD

SEQ ID NO: 19776 - protein, 9 aa, synthetic construct
GGDGKDMLT

SEQ ID NO: 19777 - protein, 9 aa, synthetic construct
GGDGKDLLD

SEQ ID NO: 19778 - protein, 9 aa, synthetic construct
GGDGKDLIT

SEQ ID NO: 19779 - protein, 9 aa, synthetic construct
GGDGKDLIG

SEQ ID NO: 19780 - protein, 9 aa, synthetic construct
GGGGLDYLS

SEQ ID NO: 19781 - protein, 9 aa, synthetic construct
GGDGKDILH

SEQ ID NO: 19782 - protein, 9 aa, synthetic construct
GGLGHDDLG

SEQ ID NO: 19783 - protein, 9 aa, synthetic construct
GGDGKDILT

SEQ ID NO: 19784 - protein, 9 aa, synthetic construct
GGDGKDILV

SEQ ID NO: 19785 - protein, 9 aa, synthetic construct
GGLGGDYLS

SEQ ID NO: 19786 - protein, 9 aa, synthetic construct
GGGGLDWFL

SEQ ID NO: 19787 - protein, 9 aa, synthetic construct
GGDGKDKLN

SEQ ID NO: 19788 - protein, 9 aa, synthetic construct
GGGGMDLLI

SEQ ID NO: 19789 - protein, 9 aa, synthetic construct
GGLGGDVLS

SEQ ID NO: 19790 - protein, 9 aa, synthetic construct
GGLGGDVLN

SEQ ID NO: 19791 - protein, 9 aa, synthetic construct
GGDGKDKLR

SEQ ID NO: 19792 - protein, 9 aa, synthetic construct
GGLGGDVIN

SEQ ID NO: 19793 - protein, 9 aa, synthetic construct
GGEGDDFLL

SEQ ID NO: 19794 - protein, 9 aa, synthetic construct
GGLGGDTVR

SEQ ID NO: 19795 - protein, 9 aa, synthetic construct
GGDGKDVLV

SEQ ID NO: 19796 - protein, 9 aa, synthetic construct
GGEGDDELW

SEQ ID NO: 19797 - protein, 9 aa, synthetic construct
GGLGIDEMS

SEQ ID NO: 19798 - protein, 9 aa, synthetic construct
GGGGNDFVQ

SEQ ID NO: 19799 - protein, 9 aa, synthetic construct
GGLGDDQLL

SEQ ID NO: 19800 - protein, 9 aa, synthetic construct
GGLGDDQLH

SEQ ID NO: 19801 - protein, 9 aa, synthetic construct
GGLGDDQLE

SEQ ID NO: 19802 - protein, 9 aa, synthetic construct
GGLGDDQIW

SEQ ID NO: 19803 - protein, 9 aa, synthetic construct
GGLGDDQIT

SEQ ID NO: 19804 - protein, 9 aa, synthetic construct
GGGGNDGFS

SEQ ID NO: 19805 - protein, 9 aa, synthetic construct
GGEGDDDLE

SEQ ID NO: 19806 - protein, 9 aa, synthetic construct
GGLGDDNLT

SEQ ID NO: 19807 - protein, 9 aa, synthetic construct
GGLGDDNLM

SEQ ID NO: 19808 - protein, 9 aa, synthetic construct
GGDGLDWVR

SEQ ID NO: 19809 - protein, 9 aa, synthetic construct
GGLGDDNIN

SEQ ID NO: 19810 - protein, 9 aa, synthetic construct
GGDGLDYIS

SEQ ID NO: 19811 - protein, 9 aa, synthetic construct
GGLGDDMLW

SEQ ID NO: 19812 - protein, 9 aa, synthetic construct
GGDGMDAAS

SEQ ID NO: 19813 - protein, 9 aa, synthetic construct
GGLGDDMLS

SEQ ID NO: 19814 - protein, 9 aa, synthetic construct
GGGGNDFVS

SEQ ID NO: 19815 - protein, 9 aa, synthetic construct
GGDGLDVLN

SEQ ID NO: 19816 - protein, 9 aa, synthetic construct
GGLGDDSLA

SEQ ID NO: 19817 - protein, 9 aa, synthetic construct
GGGGNDFVA

SEQ ID NO: 19818 - protein, 9 aa, synthetic construct
GGLGDDSIN

SEQ ID NO: 19819 - protein, 9 aa, synthetic construct
GGLGDDSIF

SEQ ID NO: 19820 - protein, 9 aa, synthetic construct
GGGGNDFLQ

SEQ ID NO: 19821 - protein, 9 aa, synthetic construct
GGLGDDRYY

SEQ ID NO: 19822 - protein, 9 aa, synthetic construct
GGLGDDRVY

SEQ ID NO: 19823 - protein, 9 aa, synthetic construct
GGLGDDRVR

SEQ ID NO: 19824 - protein, 9 aa, synthetic construct
GGLGDDRMY

SEQ ID NO: 19825 - protein, 9 aa, synthetic construct
GGLGDDRLR

SEQ ID NO: 19826 - protein, 9 aa, synthetic construct
GGLGDDRLN

SEQ ID NO: 19827 - protein, 9 aa, synthetic construct
GGDGLDTMY

SEQ ID NO: 19828 - protein, 9 aa, synthetic construct
GGLGDDRIV

SEQ ID NO: 19829 - protein, 9 aa, synthetic construct
GGGGNDFMA

SEQ ID NO: 19830 - protein, 9 aa, synthetic construct
GGEGDDDLQ

SEQ ID NO: 19831 - protein, 9 aa, synthetic construct
GGLGDDRAL

SEQ ID NO: 19832 - protein, 9 aa, synthetic construct
GGLGDDQYT

SEQ ID NO: 19833 - protein, 9 aa, synthetic construct
GGDGMDAIY

SEQ ID NO: 19834 - protein, 9 aa, synthetic construct
GGLGDDMLF

SEQ ID NO: 19835 - protein, 9 aa, synthetic construct
GGEGDDDIW

SEQ ID NO: 19836 - protein, 9 aa, synthetic construct
GGGGNDGLW

SEQ ID NO: 19837 - protein, 9 aa, synthetic construct
GGLGDDLFD

SEQ ID NO: 19838 - protein, 9 aa, synthetic construct
GGLGDDKVQ

SEQ ID NO: 19839 - protein, 9 aa, synthetic construct
GGGGNDHLE

SEQ ID NO: 19840 - protein, 9 aa, synthetic construct
GGDGMDRLF

SEQ ID NO: 19841 - protein, 9 aa, synthetic construct
GGGGNDHLH

SEQ ID NO: 19842 - protein, 9 aa, synthetic construct
GGGGNDHLK

SEQ ID NO: 19843 - protein, 9 aa, synthetic construct
GGGGNDHLL

SEQ ID NO: 19844 - protein, 9 aa, synthetic construct
GGLGDDKLE

SEQ ID NO: 19845 - protein, 9 aa, synthetic construct
GGLGDDKIF

SEQ ID NO: 19846 - protein, 9 aa, synthetic construct
GGGGNDHLS

SEQ ID NO: 19847 - protein, 9 aa, synthetic construct
GGDGMDTLA

SEQ ID NO: 19848 - protein, 9 aa, synthetic construct
GGLGDDIYG

SEQ ID NO: 19849 - protein, 9 aa, synthetic construct
GGEGDDAVF

SEQ ID NO: 19850 - protein, 9 aa, synthetic construct
GGDGMDTLI

SEQ ID NO: 19851 - protein, 9 aa, synthetic construct
GGLGDDIVN

SEQ ID NO: 19852 - protein, 9 aa, synthetic construct
GGDGMDQLI

SEQ ID NO: 19853 - protein, 9 aa, synthetic construct
GGLGDDLFL

SEQ ID NO: 19854 - protein, 9 aa, synthetic construct
GGLGDDLFQ

SEQ ID NO: 19855 - protein, 9 aa, synthetic construct
GGGGNDGVM

SEQ ID NO: 19856 - protein, 9 aa, synthetic construct
GGLGDDMID

SEQ ID NO: 19857 - protein, 9 aa, synthetic construct
GGLGDDMFF

SEQ ID NO: 19858 - protein, 9 aa, synthetic construct
GGLGDDLYR

SEQ ID NO: 19859 - protein, 9 aa, synthetic construct
GGGGNDGLY

SEQ ID NO: 19860 - protein, 9 aa, synthetic construct
GGDGMDIAD

SEQ ID NO: 19861 - protein, 9 aa, synthetic construct
GGLGDDLVV

SEQ ID NO: 19862 - protein, 9 aa, synthetic construct
GGEGDDDIR

SEQ ID NO: 19863 - protein, 9 aa, synthetic construct
GGGGNDHID

SEQ ID NO: 19864 - protein, 9 aa, synthetic construct
GGEGDDDIK

SEQ ID NO: 19865 - protein, 9 aa, synthetic construct
GGLGDDLLX

SEQ ID NO: 19866 - protein, 9 aa, synthetic construct
GGLGDDLLM

SEQ ID NO: 19867 - protein, 9 aa, synthetic construct
GGLGDDLLG

SEQ ID NO: 19868 - protein, 9 aa, synthetic construct
GGLGDDLLA

SEQ ID NO: 19869 - protein, 9 aa, synthetic construct
GGLGDDLIR

SEQ ID NO: 19870 - protein, 9 aa, synthetic construct
GGLGDDSIV

SEQ ID NO: 19871 - protein, 9 aa, synthetic construct
GGLGDDSLE

SEQ ID NO: 19872 - protein, 9 aa, synthetic construct
GGEGDDELV

SEQ ID NO: 19873 - protein, 9 aa, synthetic construct
GGLGEDFLD

SEQ ID NO: 19874 - protein, 9 aa, synthetic construct
GGDGLDFLY

SEQ ID NO: 19875 - protein, 9 aa, synthetic construct
GGDGLDFVN

SEQ ID NO: 19876 - protein, 9 aa, synthetic construct
GGLGDDYVR

SEQ ID NO: 19877 - protein, 9 aa, synthetic construct
GGGGNDEIA

SEQ ID NO: 19878 - protein, 9 aa, synthetic construct
GGLGDDYLV

SEQ ID NO: 19879 - protein, 9 aa, synthetic construct
GGGGNDEIE

SEQ ID NO: 19880 - protein, 9 aa, synthetic construct
GGDGLDIFV

SEQ ID NO: 19881 - protein, 9 aa, synthetic construct
GGLGDDYLQ

SEQ ID NO: 19882 - protein, 9 aa, synthetic construct
GGDGLDILI

SEQ ID NO: 19883 - protein, 9 aa, synthetic construct
GGGGNDEIL

SEQ ID NO: 19884 - protein, 9 aa, synthetic construct
GGGGNDEIN

SEQ ID NO: 19885 - protein, 9 aa, synthetic construct
GGLGDDYFI

SEQ ID NO: 19886 - protein, 9 aa, synthetic construct
GGGGNDEIQ

SEQ ID NO: 19887 - protein, 9 aa, synthetic construct
GGDGLDILY

SEQ ID NO: 19888 - protein, 9 aa, synthetic construct
GGLGDDWLF

SEQ ID NO: 19889 - protein, 9 aa, synthetic construct
GGDGLDFLD

SEQ ID NO: 19890 - protein, 9 aa, synthetic construct
GGLGEDHFI

SEQ ID NO: 19891 - protein, 9 aa, synthetic construct
GGLGDDSLR

SEQ ID NO: 19892 - protein, 9 aa, synthetic construct
GGGGNDDLT

SEQ ID NO: 19893 - protein, 9 aa, synthetic construct
GGGGNDDID

SEQ ID NO: 19894 - protein, 9 aa, synthetic construct
GGLGEDSLI

SEQ ID NO: 19895 - protein, 9 aa, synthetic construct
GGGGNDDIN

SEQ ID NO: 19896 - protein, 9 aa, synthetic construct
GGLGEDSLD

SEQ ID NO: 19897 - protein, 9 aa, synthetic construct
GGDGKDWLT

SEQ ID NO: 19898 - protein, 9 aa, synthetic construct
GGLGEDSFY

SEQ ID NO: 19899 - protein, 9 aa, synthetic construct
GGDGKDYFV

SEQ ID NO: 19900 - protein, 9 aa, synthetic construct
GGEGDDELT

SEQ ID NO: 19901 - protein, 9 aa, synthetic construct
GGDGKDYLS

SEQ ID NO: 19902 - protein, 9 aa, synthetic construct
GGLGEDLLE

SEQ ID NO: 19903 - protein, 9 aa, synthetic construct
GGGGNDDLH

SEQ ID NO: 19904 - protein, 9 aa, synthetic construct
GGDGLDEIS

SEQ ID NO: 19905 - protein, 9 aa, synthetic construct
GGEGDDELK

SEQ ID NO: 19906 - protein, 9 aa, synthetic construct
GGGGNDDLR

SEQ ID NO: 19907 - protein, 9 aa, synthetic construct
GGDGLDFAD

SEQ ID NO: 19908 - protein, 9 aa, synthetic construct
GGLGDDWLD

SEQ ID NO: 19909 - protein, 9 aa, synthetic construct
GGEGDDEIT

SEQ ID NO: 19910 - protein, 9 aa, synthetic construct
GGDGLDLLL

SEQ ID NO: 19911 - protein, 9 aa, synthetic construct
GGLGDDWFD

SEQ ID NO: 19912 - protein, 9 aa, synthetic construct
GGLGDDTLW

SEQ ID NO: 19913 - protein, 9 aa, synthetic construct
GGLGDDTLK

SEQ ID NO: 19914 - protein, 9 aa, synthetic construct
GGDGLDSLD

SEQ ID NO: 19915 - protein, 9 aa, synthetic construct
GGLGDDTIH

SEQ ID NO: 19916 - protein, 9 aa, synthetic construct
GGLGDDTIG

SEQ ID NO: 19917 - protein, 9 aa, synthetic construct
GGGGNDFIV

SEQ ID NO: 19918 - protein, 9 aa, synthetic construct
GGLGDDTFA

SEQ ID NO: 19919 - protein, 9 aa, synthetic construct
GGLGDDTAI

SEQ ID NO: 19920 - protein, 9 aa, synthetic construct
GGLGDDSYQ

SEQ ID NO: 19921 - protein, 9 aa, synthetic construct
GGLGDDSYK

SEQ ID NO: 19922 - protein, 9 aa, synthetic construct
GGLGDDSYI

SEQ ID NO: 19923 - protein, 9 aa, synthetic construct
GGDGLDTLA

SEQ ID NO: 19924 - protein, 9 aa, synthetic construct
GGLGDDSML

SEQ ID NO: 19925 - protein, 9 aa, synthetic construct
GGDGLDTLE

SEQ ID NO: 19926 - protein, 9 aa, synthetic construct
GGDGLDTLH

SEQ ID NO: 19927 - protein, 9 aa, synthetic construct
GGGGNDFIE

SEQ ID NO: 19928 - protein, 9 aa, synthetic construct
GGDGLDRMI

SEQ ID NO: 19929 - protein, 9 aa, synthetic construct
GGLGDDTVI

SEQ ID NO: 19930 - protein, 9 aa, synthetic construct
GGLGDDVLW

SEQ ID NO: 19931 - protein, 9 aa, synthetic construct
GGGGNDELI

SEQ ID NO: 19932 - protein, 9 aa, synthetic construct
GGGGNDELQ

SEQ ID NO: 19933 - protein, 9 aa, synthetic construct
GGLGDDVVI

SEQ ID NO: 19934 - protein, 9 aa, synthetic construct
GGLGDDVMT

SEQ ID NO: 19935 - protein, 9 aa, synthetic construct
GGLGDDVME

SEQ ID NO: 19936 - protein, 9 aa, synthetic construct
GGLGDDVMA

SEQ ID NO: 19937 - protein, 9 aa, synthetic construct
GGGGNDEMH

SEQ ID NO: 19938 - protein, 9 aa, synthetic construct
GGLGDDTVV

SEQ ID NO: 19939 - protein, 9 aa, synthetic construct
GGLGDDVIL

SEQ ID NO: 19940 - protein, 9 aa, synthetic construct
GGLGDDVFR

SEQ ID NO: 19941 - protein, 9 aa, synthetic construct
GGLGDDVFN

SEQ ID NO: 19942 - protein, 9 aa, synthetic construct
GGLGDDVFE

SEQ ID NO: 19943 - protein, 9 aa, synthetic construct
GGGGNDFFS

SEQ ID NO: 19944 - protein, 9 aa, synthetic construct
GGLGDDTYH

SEQ ID NO: 19945 - protein, 9 aa, synthetic construct
GGLGIDELT

SEQ ID NO: 19946 - protein, 9 aa, synthetic construct
GGDGIDTVK

SEQ ID NO: 19947 - protein, 9 aa, synthetic construct
GGDGNDWIE

SEQ ID NO: 19948 - protein, 9 aa, synthetic construct
GGEGDDKIY

SEQ ID NO: 19949 - protein, 9 aa, synthetic construct
GGLGNDNLQ

SEQ ID NO: 19950 - protein, 9 aa, synthetic construct
GGLGNDNLG

SEQ ID NO: 19951 - protein, 9 aa, synthetic construct
GGLGNDNLF

SEQ ID NO: 19952 - protein, 9 aa, synthetic construct
GGDGHDRIE

SEQ ID NO: 19953 - protein, 9 aa, synthetic construct
GGLGNDMYR

SEQ ID NO: 19954 - protein, 9 aa, synthetic construct
GGDGHDRLE

SEQ ID NO: 19955 - protein, 9 aa, synthetic construct
GGLGNDMLQ

SEQ ID NO: 19956 - protein, 9 aa, synthetic construct
GGLGNDMLE

SEQ ID NO: 19957 - protein, 9 aa, synthetic construct
GGLGNDMID

SEQ ID NO: 19958 - protein, 9 aa, synthetic construct
GGDGHDRLI

SEQ ID NO: 19959 - protein, 9 aa, synthetic construct
GGLGNDLYL

SEQ ID NO: 19960 - protein, 9 aa, synthetic construct
GGLGNDLVL

SEQ ID NO: 19961 - protein, 9 aa, synthetic construct
GGDGHDRLT

SEQ ID NO: 19962 - protein, 9 aa, synthetic construct
GGDGHDRLV

SEQ ID NO: 19963 - protein, 9 aa, synthetic construct
GGLGNDLMK

SEQ ID NO: 19964 - protein, 9 aa, synthetic construct
GGGGKDKLL

SEQ ID NO: 19965 - protein, 9 aa, synthetic construct
GGLGNDNYV

SEQ ID NO: 19966 - protein, 9 aa, synthetic construct
GGEGDDKLE

SEQ ID NO: 19967 - protein, 9 aa, synthetic construct
GGLGNDQFN

SEQ ID NO: 19968 - protein, 9 aa, synthetic construct
GGGGKDKII

SEQ ID NO: 19969 - protein, 9 aa, synthetic construct
GGGGKDKIK

SEQ ID NO: 19970 - protein, 9 aa, synthetic construct
GGDGHDQIF

SEQ ID NO: 19971 - protein, 9 aa, synthetic construct
GGLGNDQMF

SEQ ID NO: 19972 - protein, 9 aa, synthetic construct
GGGGKDKIS

SEQ ID NO: 19973 - protein, 9 aa, synthetic construct
GGDGHDQLD

SEQ ID NO: 19974 - protein, 9 aa, synthetic construct
GGLGNDQLI

SEQ ID NO: 19975 - protein, 9 aa, synthetic construct
GGLGNDQLE

SEQ ID NO: 19976 - protein, 9 aa, synthetic construct
GGDGHDQLN

SEQ ID NO: 19977 - protein, 9 aa, synthetic construct
GGLGNDQIQ

SEQ ID NO: 19978 - protein, 9 aa, synthetic construct
GGLGNDQIL

SEQ ID NO: 19979 - protein, 9 aa, synthetic construct
GGLGNDQIH

SEQ ID NO: 19980 - protein, 9 aa, synthetic construct
GGLGNDQIE

SEQ ID NO: 19981 - protein, 9 aa, synthetic construct
GGLGNDQID

SEQ ID NO: 19982 - protein, 9 aa, synthetic construct
GGDGHDQLT

SEQ ID NO: 19983 - protein, 9 aa, synthetic construct
GGLGNDLMF

SEQ ID NO: 19984 - protein, 9 aa, synthetic construct
GGLGNDLME

SEQ ID NO: 19985 - protein, 9 aa, synthetic construct
GGLGNDLLW

SEQ ID NO: 19986 - protein, 9 aa, synthetic construct
GGLGNDLLA

SEQ ID NO: 19987 - protein, 9 aa, synthetic construct
GGLGNDIYA

SEQ ID NO: 19988 - protein, 9 aa, synthetic construct
GGDGHDSLT

SEQ ID NO: 19989 - protein, 9 aa, synthetic construct
GGLGNDIVK

SEQ ID NO: 19990 - protein, 9 aa, synthetic construct
GGLGNDIMR

SEQ ID NO: 19991 - protein, 9 aa, synthetic construct
GGEGDDIYL

SEQ ID NO: 19992 - protein, 9 aa, synthetic construct
GGLGNDILH

SEQ ID NO: 19993 - protein, 9 aa, synthetic construct
GGLGNDILG

SEQ ID NO: 19994 - protein, 9 aa, synthetic construct
GGLGNDILE

SEQ ID NO: 19995 - protein, 9 aa, synthetic construct
GGLGNDIIT

SEQ ID NO: 19996 - protein, 9 aa, synthetic construct
GGLGNDIIS

SEQ ID NO: 19997 - protein, 9 aa, synthetic construct
GGLGNDIIR

SEQ ID NO: 19998 - protein, 9 aa, synthetic construct
GGLGNDIII

SEQ ID NO: 19999 - protein, 9 aa, synthetic construct
GGLGNDIIH

SEQ ID NO: 20000 - protein, 9 aa, synthetic construct
GGGGKDLMT

SEQ ID NO: 20001 - protein, 9 aa, synthetic construct
GGEGDDIVY

SEQ ID NO: 20002 - protein, 9 aa, synthetic construct
GGLGNDIYQ

SEQ ID NO: 20003 - protein, 9 aa, synthetic construct
GGLGNDKID

SEQ ID NO: 20004 - protein, 9 aa, synthetic construct
GGDGHDSLF

SEQ ID NO: 20005 - protein, 9 aa, synthetic construct
GGLGNDLFD

SEQ ID NO: 20006 - protein, 9 aa, synthetic construct
GGLGNDLIW

SEQ ID NO: 20007 - protein, 9 aa, synthetic construct
GGLGNDLIQ

SEQ ID NO: 20008 - protein, 9 aa, synthetic construct
GGEGDDIYY

SEQ ID NO: 20009 - protein, 9 aa, synthetic construct
GGLGNDLFY

SEQ ID NO: 20010 - protein, 9 aa, synthetic construct
GGLGNDLFV

SEQ ID NO: 20011 - protein, 9 aa, synthetic construct
GGLGNDLFS

SEQ ID NO: 20012 - protein, 9 aa, synthetic construct
GGDGHDSFG

SEQ ID NO: 20013 - protein, 9 aa, synthetic construct
GGLGNDKIT

SEQ ID NO: 20014 - protein, 9 aa, synthetic construct
GGLGNDLAE

SEQ ID NO: 20015 - protein, 9 aa, synthetic construct
GGGGKDLLL

SEQ ID NO: 20016 - protein, 9 aa, synthetic construct
GGDGHDSLA

SEQ ID NO: 20017 - protein, 9 aa, synthetic construct
GGLGNDKLN

SEQ ID NO: 20018 - protein, 9 aa, synthetic construct
GGLGNDKLH

SEQ ID NO: 20019 - protein, 9 aa, synthetic construct
GGLGNDKLE

SEQ ID NO: 20020 - protein, 9 aa, synthetic construct
GGDGHDNLV

SEQ ID NO: 20021 - protein, 9 aa, synthetic construct
GGGGKDILV

SEQ ID NO: 20022 - protein, 9 aa, synthetic construct
GGGGKDMLD

SEQ ID NO: 20023 - protein, 9 aa, synthetic construct
GGLGNDVMS

SEQ ID NO: 20024 - protein, 9 aa, synthetic construct
GGLGNDVLW

SEQ ID NO: 20025 - protein, 9 aa, synthetic construct
GGLGNDVLG

SEQ ID NO: 20026 - protein, 9 aa, synthetic construct
GGDGHDILK

SEQ ID NO: 20027 - protein, 9 aa, synthetic construct
GGLGNDVFS

SEQ ID NO: 20028 - protein, 9 aa, synthetic construct
GGLGNDVFH

SEQ ID NO: 20029 - protein, 9 aa, synthetic construct
GGLGNDVFE

SEQ ID NO: 20030 - protein, 9 aa, synthetic construct
GGGGKDDLS

SEQ ID NO: 20031 - protein, 9 aa, synthetic construct
GGLGNDVAN

SEQ ID NO: 20032 - protein, 9 aa, synthetic construct
GGLGNDTYS

SEQ ID NO: 20033 - protein, 9 aa, synthetic construct
GGLGNDTYE

SEQ ID NO: 20034 - protein, 9 aa, synthetic construct
GGDGHDIMD

SEQ ID NO: 20035 - protein, 9 aa, synthetic construct
GGLGNDTVR

SEQ ID NO: 20036 - protein, 9 aa, synthetic construct
GGEGDDKMR

SEQ ID NO: 20037 - protein, 9 aa, synthetic construct
GGLGNDTVI

SEQ ID NO: 20038 - protein, 9 aa, synthetic construct
GGDGHDIMS

SEQ ID NO: 20039 - protein, 9 aa, synthetic construct
GGLGNDVMD

SEQ ID NO: 20040 - protein, 9 aa, synthetic construct
GGEGDDKVF

SEQ ID NO: 20041 - protein, 9 aa, synthetic construct
GGGGKDILT

SEQ ID NO: 20042 - protein, 9 aa, synthetic construct
GGGGKDAVN

SEQ ID NO: 20043 - protein, 9 aa, synthetic construct
GGEGDDLFE

SEQ ID NO: 20044 - protein, 9 aa, synthetic construct
GGLGNDYLA

SEQ ID NO: 20045 - protein, 9 aa, synthetic construct
GGDGHDFIH

SEQ ID NO: 20046 - protein, 9 aa, synthetic construct
GGLGNDYIS

SEQ ID NO: 20047 - protein, 9 aa, synthetic construct
GGDGHDFLF

SEQ ID NO: 20048 - protein, 9 aa, synthetic construct
GGLGNDYIA

SEQ ID NO: 20049 - protein, 9 aa, synthetic construct
GGGGIDYLS

SEQ ID NO: 20050 - protein, 9 aa, synthetic construct
GGGGIDYVL

SEQ ID NO: 20051 - protein, 9 aa, synthetic construct
GGLGNDWLL

SEQ ID NO: 20052 - protein, 9 aa, synthetic construct
GGLGNDWLG

SEQ ID NO: 20053 - protein, 9 aa, synthetic construct
GGEGDDLAR

SEQ ID NO: 20054 - protein, 9 aa, synthetic construct
GGDGHDHLF

SEQ ID NO: 20055 - protein, 9 aa, synthetic construct
GGGGKDALH

SEQ ID NO: 20056 - protein, 9 aa, synthetic construct
GGLGNDVYS

SEQ ID NO: 20057 - protein, 9 aa, synthetic construct
GGGGKDALY

SEQ ID NO: 20058 - protein, 9 aa, synthetic construct
GGLGNDTVE

SEQ ID NO: 20059 - protein, 9 aa, synthetic construct
GGLGNDTME

SEQ ID NO: 20060 - protein, 9 aa, synthetic construct
GGLGNDTFY

SEQ ID NO: 20061 - protein, 9 aa, synthetic construct
GGDGHDKLH

SEQ ID NO: 20062 - protein, 9 aa, synthetic construct
GGDGHDLIQ

SEQ ID NO: 20063 - protein, 9 aa, synthetic construct
GGLGNDSFV

SEQ ID NO: 20064 - protein, 9 aa, synthetic construct
GGLGNDSFR

SEQ ID NO: 20065 - protein, 9 aa, synthetic construct
GGEGDDKLM

SEQ ID NO: 20066 - protein, 9 aa, synthetic construct
GGLGNDRYY

SEQ ID NO: 20067 - protein, 9 aa, synthetic construct
GGLGNDRYQ

SEQ ID NO: 20068 - protein, 9 aa, synthetic construct
GGLGNDRVY

SEQ ID NO: 20069 - protein, 9 aa, synthetic construct
GGLGNDRVD

SEQ ID NO: 20070 - protein, 9 aa, synthetic construct
GGLGNDRMN

SEQ ID NO: 20071 - protein, 9 aa, synthetic construct
GGGGKDIFV

SEQ ID NO: 20072 - protein, 9 aa, synthetic construct
GGDGHDMLD

SEQ ID NO: 20073 - protein, 9 aa, synthetic construct
GGLGNDRLR

SEQ ID NO: 20074 - protein, 9 aa, synthetic construct
GGLGNDRIN

SEQ ID NO: 20075 - protein, 9 aa, synthetic construct
GGDGHDMLW

SEQ ID NO: 20076 - protein, 9 aa, synthetic construct
GGGGKDILS

SEQ ID NO: 20077 - protein, 9 aa, synthetic construct
GGLGNDSIY

SEQ ID NO: 20078 - protein, 9 aa, synthetic construct
GGLGNDSLH

SEQ ID NO: 20079 - protein, 9 aa, synthetic construct
GGLGNDSLM

SEQ ID NO: 20080 - protein, 9 aa, synthetic construct
GGLGNDTAN

SEQ ID NO: 20081 - protein, 9 aa, synthetic construct
GGGGKDEIS

SEQ ID NO: 20082 - protein, 9 aa, synthetic construct
GGLGNDTFG

SEQ ID NO: 20083 - protein, 9 aa, synthetic construct
GGLGNDTFD

SEQ ID NO: 20084 - protein, 9 aa, synthetic construct
GGDGHDKLW

SEQ ID NO: 20085 - protein, 9 aa, synthetic construct
GGLGNDTAY

SEQ ID NO: 20086 - protein, 9 aa, synthetic construct
GGLGNDTAT

SEQ ID NO: 20087 - protein, 9 aa, synthetic construct
GGLGNDSYW

SEQ ID NO: 20088 - protein, 9 aa, synthetic construct
GGDGHDLIL

SEQ ID NO: 20089 - protein, 9 aa, synthetic construct
GGLGNDSYT

SEQ ID NO: 20090 - protein, 9 aa, synthetic construct
GGLGNDSVM

SEQ ID NO: 20091 - protein, 9 aa, synthetic construct
GGLGNDSVL

SEQ ID NO: 20092 - protein, 9 aa, synthetic construct
GGLGNDSMV

SEQ ID NO: 20093 - protein, 9 aa, synthetic construct
GGDGHDLII

SEQ ID NO: 20094 - protein, 9 aa, synthetic construct
GGLGNDSLW

SEQ ID NO: 20095 - protein, 9 aa, synthetic construct
GGGGKDMIR

SEQ ID NO: 20096 - protein, 9 aa, synthetic construct
GGLGNDIAT

SEQ ID NO: 20097 - protein, 9 aa, synthetic construct
GGGGLDMLD

SEQ ID NO: 20098 - protein, 9 aa, synthetic construct
GGLGKDTLD

SEQ ID NO: 20099 - protein, 9 aa, synthetic construct
GGEGDDIFV

SEQ ID NO: 20100 - protein, 9 aa, synthetic construct
GGLGKDTIR

SEQ ID NO: 20101 - protein, 9 aa, synthetic construct
GGLGKDTIA

SEQ ID NO: 20102 - protein, 9 aa, synthetic construct
GGLGKDTFI

SEQ ID NO: 20103 - protein, 9 aa, synthetic construct
GGLGKDTAD

SEQ ID NO: 20104 - protein, 9 aa, synthetic construct
GGLGKDSLK

SEQ ID NO: 20105 - protein, 9 aa, synthetic construct
GGGGKDVLS

SEQ ID NO: 20106 - protein, 9 aa, synthetic construct
GGLGKDRLD

SEQ ID NO: 20107 - protein, 9 aa, synthetic construct
GGLGKDQLT

SEQ ID NO: 20108 - protein, 9 aa, synthetic construct
GGLGKDQLS

SEQ ID NO: 20109 - protein, 9 aa, synthetic construct
GGDGIDRAS

SEQ ID NO: 20110 - protein, 9 aa, synthetic construct
GGDGIDRIQ

SEQ ID NO: 20111 - protein, 9 aa, synthetic construct
GGLGKDNLD

SEQ ID NO: 20112 - protein, 9 aa, synthetic construct
GGGGKDYIK

SEQ ID NO: 20113 - protein, 9 aa, synthetic construct
GGLGKDMLY

SEQ ID NO: 20114 - protein, 9 aa, synthetic construct
GGGGKDVLL

SEQ ID NO: 20115 - protein, 9 aa, synthetic construct
GGLGKDTLE

SEQ ID NO: 20116 - protein, 9 aa, synthetic construct
GGLGLDKLA

SEQ ID NO: 20117 - protein, 9 aa, synthetic construct
GGGGKDVLK

SEQ ID NO: 20118 - protein, 9 aa, synthetic construct
GGLGLDFLD

SEQ ID NO: 20119 - protein, 9 aa, synthetic construct
GGGGKDVFI

SEQ ID NO: 20120 - protein, 9 aa, synthetic construct
GGDGIDLID

SEQ ID NO: 20121 - protein, 9 aa, synthetic construct
GGGGKDVFV

SEQ ID NO: 20122 - protein, 9 aa, synthetic construct
GGLGKDYLT

SEQ ID NO: 20123 - protein, 9 aa, synthetic construct
GGDGIDLLA

SEQ ID NO: 20124 - protein, 9 aa, synthetic construct
GGDGIDLLL

SEQ ID NO: 20125 - protein, 9 aa, synthetic construct
GGLGKDVLK

SEQ ID NO: 20126 - protein, 9 aa, synthetic construct
GGLGKDVFV

SEQ ID NO: 20127 - protein, 9 aa, synthetic construct
GGLGKDVFL

SEQ ID NO: 20128 - protein, 9 aa, synthetic construct
GGDGIDLLS

SEQ ID NO: 20129 - protein, 9 aa, synthetic construct
GGLGKDTYV

SEQ ID NO: 20130 - protein, 9 aa, synthetic construct
GGGGKDVLE

SEQ ID NO: 20131 - protein, 9 aa, synthetic construct
GGLGKDTMA

SEQ ID NO: 20132 - protein, 9 aa, synthetic construct
GGLGKDTLI

SEQ ID NO: 20133 - protein, 9 aa, synthetic construct
GGLGKDLMI

SEQ ID NO: 20134 - protein, 9 aa, synthetic construct
GGGGKDYLI

SEQ ID NO: 20135 - protein, 9 aa, synthetic construct
GGEGDDHYY

SEQ ID NO: 20136 - protein, 9 aa, synthetic construct
GGGGLDALS

SEQ ID NO: 20137 - protein, 9 aa, synthetic construct
GGLGIDTLN

SEQ ID NO: 20138 - protein, 9 aa, synthetic construct
GGLGIDTLD

SEQ ID NO: 20139 - protein, 9 aa, synthetic construct
GGEGDDHLL

SEQ ID NO: 20140 - protein, 9 aa, synthetic construct
GGDGIDTIH

SEQ ID NO: 20141 - protein, 9 aa, synthetic construct
GGDGIDTIV

SEQ ID NO: 20142 - protein, 9 aa, synthetic construct
GGDGIDTIW

SEQ ID NO: 20143 - protein, 9 aa, synthetic construct
GGDGIDTLE

SEQ ID NO: 20144 - protein, 9 aa, synthetic construct
GGDGIDTLG

SEQ ID NO: 20145 - protein, 9 aa, synthetic construct
GGLGIDRLL

SEQ ID NO: 20146 - protein, 9 aa, synthetic construct
GGDGIDTLQ

SEQ ID NO: 20147 - protein, 9 aa, synthetic construct
GGDGIDTLT

SEQ ID NO: 20148 - protein, 9 aa, synthetic construct
GGLGIDNIH

SEQ ID NO: 20149 - protein, 9 aa, synthetic construct
GGLGIDKME

SEQ ID NO: 20150 - protein, 9 aa, synthetic construct
GGEGDDHLF

SEQ ID NO: 20151 - protein, 9 aa, synthetic construct
GGLGIDIMV

SEQ ID NO: 20152 - protein, 9 aa, synthetic construct
GGLGIDTLQ

SEQ ID NO: 20153 - protein, 9 aa, synthetic construct
GGLGIDTLY

SEQ ID NO: 20154 - protein, 9 aa, synthetic construct
GGLGIDTMA

SEQ ID NO: 20155 - protein, 9 aa, synthetic construct
GGGGLDFIF

SEQ ID NO: 20156 - protein, 9 aa, synthetic construct
GGLGKDKLT

SEQ ID NO: 20157 - protein, 9 aa, synthetic construct
GGDGIDSID

SEQ ID NO: 20158 - protein, 9 aa, synthetic construct
GGLGKDILS

SEQ ID NO: 20159 - protein, 9 aa, synthetic construct
GGLGKDILN

SEQ ID NO: 20160 - protein, 9 aa, synthetic construct
GGDGIDSLL

SEQ ID NO: 20161 - protein, 9 aa, synthetic construct
GGLGKDELT

SEQ ID NO: 20162 - protein, 9 aa, synthetic construct
GGDGIDSLT

SEQ ID NO: 20163 - protein, 9 aa, synthetic construct
GGGGLDKFL

SEQ ID NO: 20164 - protein, 9 aa, synthetic construct
GGGGLDFVD

SEQ ID NO: 20165 - protein, 9 aa, synthetic construct
GGLGKDALA

SEQ ID NO: 20166 - protein, 9 aa, synthetic construct
GGLGIDWLD

SEQ ID NO: 20167 - protein, 9 aa, synthetic construct
GGLGIDVLV

SEQ ID NO: 20168 - protein, 9 aa, synthetic construct
GGDGIDTAF

SEQ ID NO: 20169 - protein, 9 aa, synthetic construct
GGEGDDHLN

SEQ ID NO: 20170 - protein, 9 aa, synthetic construct
GGLGLDILQ

SEQ ID NO: 20171 - protein, 9 aa, synthetic construct
GGDGIDILT

SEQ ID NO: 20172 - protein, 9 aa, synthetic construct
GGDGHDTIF

SEQ ID NO: 20173 - protein, 9 aa, synthetic construct
GGLGNDFLA

SEQ ID NO: 20174 - protein, 9 aa, synthetic construct
GGLGNDFIG

SEQ ID NO: 20175 - protein, 9 aa, synthetic construct
GGLGNDFIA

SEQ ID NO: 20176 - protein, 9 aa, synthetic construct
GGLGNDFFA

SEQ ID NO: 20177 - protein, 9 aa, synthetic construct
GGLGNDEYS

SEQ ID NO: 20178 - protein, 9 aa, synthetic construct
GGLGNDEMI

SEQ ID NO: 20179 - protein, 9 aa, synthetic construct
GGLGNDELN

SEQ ID NO: 20180 - protein, 9 aa, synthetic construct
GGLGNDELI

SEQ ID NO: 20181 - protein, 9 aa, synthetic construct
GGLGNDEII

SEQ ID NO: 20182 - protein, 9 aa, synthetic construct
GGEGDDIVE

SEQ ID NO: 20183 - protein, 9 aa, synthetic construct
GGEGDDIVD

SEQ ID NO: 20184 - protein, 9 aa, synthetic construct
GGLGNDDME

SEQ ID NO: 20185 - protein, 9 aa, synthetic construct
GGDGHDVIW

SEQ ID NO: 20186 - protein, 9 aa, synthetic construct
GGDGHDVIY

SEQ ID NO: 20187 - protein, 9 aa, synthetic construct
GGDGHDVLF

SEQ ID NO: 20188 - protein, 9 aa, synthetic construct
GGDGHDVLK

SEQ ID NO: 20189 - protein, 9 aa, synthetic construct
GGGGKDQFV

SEQ ID NO: 20190 - protein, 9 aa, synthetic construct
GGLGNDFLF

SEQ ID NO: 20191 - protein, 9 aa, synthetic construct
GGGGKDTMT

SEQ ID NO: 20192 - protein, 9 aa, synthetic construct
GGLGNDFLK

SEQ ID NO: 20193 - protein, 9 aa, synthetic construct
GGDGHDTIL

SEQ ID NO: 20194 - protein, 9 aa, synthetic construct
GGDGHDTIY

SEQ ID NO: 20195 - protein, 9 aa, synthetic construct
GGDGHDTLA

SEQ ID NO: 20196 - protein, 9 aa, synthetic construct
GGLGNDHLF

SEQ ID NO: 20197 - protein, 9 aa, synthetic construct
GGLGNDHLA

SEQ ID NO: 20198 - protein, 9 aa, synthetic construct
GGDGHDTLF

SEQ ID NO: 20199 - protein, 9 aa, synthetic construct
GGLGNDHIF

SEQ ID NO: 20200 - protein, 9 aa, synthetic construct
GGLGNDHID

SEQ ID NO: 20201 - protein, 9 aa, synthetic construct
GGLGNDGYV

SEQ ID NO: 20202 - protein, 9 aa, synthetic construct
GGGGKDNLD

SEQ ID NO: 20203 - protein, 9 aa, synthetic construct
GGLGNDGLS

SEQ ID NO: 20204 - protein, 9 aa, synthetic construct
GGLGNDFVW

SEQ ID NO: 20205 - protein, 9 aa, synthetic construct
GGDGHDTLQ

SEQ ID NO: 20206 - protein, 9 aa, synthetic construct
GGLGNDFMS

SEQ ID NO: 20207 - protein, 9 aa, synthetic construct
GGDGHDTLW

SEQ ID NO: 20208 - protein, 9 aa, synthetic construct
GGDGHDVLL

SEQ ID NO: 20209 - protein, 9 aa, synthetic construct
GGEGDDIMS

SEQ ID NO: 20210 - protein, 9 aa, synthetic construct
GGDGHDVLY

SEQ ID NO: 20211 - protein, 9 aa, synthetic construct
GGLGNDAML

SEQ ID NO: 20212 - protein, 9 aa, synthetic construct
GGLGLDTLR

SEQ ID NO: 20213 - protein, 9 aa, synthetic construct
GGLGLDTLG

SEQ ID NO: 20214 - protein, 9 aa, synthetic construct
GGLGLDTLF

SEQ ID NO: 20215 - protein, 9 aa, synthetic construct
GGLGLDTLD

SEQ ID NO: 20216 - protein, 9 aa, synthetic construct
GGGGKDTIH

SEQ ID NO: 20217 - protein, 9 aa, synthetic construct
GGDGIDEVF

SEQ ID NO: 20218 - protein, 9 aa, synthetic construct
GGLGLDTIF

SEQ ID NO: 20219 - protein, 9 aa, synthetic construct
GGLGLDTAS

SEQ ID NO: 20220 - protein, 9 aa, synthetic construct
GGDGIDFAI

SEQ ID NO: 20221 - protein, 9 aa, synthetic construct
GGLGLDSLT

SEQ ID NO: 20222 - protein, 9 aa, synthetic construct
GGGGKDTIT

SEQ ID NO: 20223 - protein, 9 aa, synthetic construct
GGGGKDTLF

SEQ ID NO: 20224 - protein, 9 aa, synthetic construct
GGLGLDRLF

SEQ ID NO: 20225 - protein, 9 aa, synthetic construct
GGGGKDTLS

SEQ ID NO: 20226 - protein, 9 aa, synthetic construct
GGLGLDLLT

SEQ ID NO: 20227 - protein, 9 aa, synthetic construct
GGGGKDTFR

SEQ ID NO: 20228 - protein, 9 aa, synthetic construct
GGDGIDEFT

SEQ ID NO: 20229 - protein, 9 aa, synthetic construct
GGDGIDAVS

SEQ ID NO: 20230 - protein, 9 aa, synthetic construct
GGDGHDWYY

SEQ ID NO: 20231 - protein, 9 aa, synthetic construct
GGLGNDALV

SEQ ID NO: 20232 - protein, 9 aa, synthetic construct
GGDGHDVVY

SEQ ID NO: 20233 - protein, 9 aa, synthetic construct
GGGGKDRLG

SEQ ID NO: 20234 - protein, 9 aa, synthetic construct
GGLGNDALG

SEQ ID NO: 20235 - protein, 9 aa, synthetic construct
GGLGNDAIT

SEQ ID NO: 20236 - protein, 9 aa, synthetic construct
GGLGNDAFD

SEQ ID NO: 20237 - protein, 9 aa, synthetic construct
GGLGMDVLL

SEQ ID NO: 20238 - protein, 9 aa, synthetic construct
GGLGLDVLD

SEQ ID NO: 20239 - protein, 9 aa, synthetic construct
GGLGMDTLT

SEQ ID NO: 20240 - protein, 9 aa, synthetic construct
GGDGHDYLD

SEQ ID NO: 20241 - protein, 9 aa, synthetic construct
GGLGMDSLD

SEQ ID NO: 20242 - protein, 9 aa, synthetic construct
GGLGMDLLT

SEQ ID NO: 20243 - protein, 9 aa, synthetic construct
GGGGKDSLT

SEQ ID NO: 20244 - protein, 9 aa, synthetic construct
GGDGIDAAR

SEQ ID NO: 20245 - protein, 9 aa, synthetic construct
GGLGDDIMN

SEQ ID NO: 20246 - protein, 9 aa, synthetic construct
GGLGDDIMM

SEQ ID NO: 20247 - protein, 9 aa, synthetic construct
GGDGMDTLT

SEQ ID NO: 20248 - protein, 9 aa, synthetic construct
GGKGNDLLF

SEQ ID NO: 20249 - protein, 9 aa, synthetic construct
GGKGNDLIS

SEQ ID NO: 20250 - protein, 9 aa, synthetic construct
GGKGNDLIL

SEQ ID NO: 20251 - protein, 9 aa, synthetic construct
GGKGNDLFI

SEQ ID NO: 20252 - protein, 9 aa, synthetic construct
GGKGNDKLT

SEQ ID NO: 20253 - protein, 9 aa, synthetic construct
GGKGNDKLA

SEQ ID NO: 20254 - protein, 9 aa, synthetic construct
GGKGNDKIY

SEQ ID NO: 20255 - protein, 9 aa, synthetic construct
GGKGNDKIW

SEQ ID NO: 20256 - protein, 9 aa, synthetic construct
GGKGNDKIL

SEQ ID NO: 20257 - protein, 9 aa, synthetic construct
GGKGNDKID

SEQ ID NO: 20258 - protein, 9 aa, synthetic construct
GGDGNDQMH

SEQ ID NO: 20259 - protein, 9 aa, synthetic construct
GGGGNDNMS

SEQ ID NO: 20260 - protein, 9 aa, synthetic construct
GGDGNDQMS

SEQ ID NO: 20261 - protein, 9 aa, synthetic construct
GGEGADWIE

SEQ ID NO: 20262 - protein, 9 aa, synthetic construct
GGKGNDIMT

SEQ ID NO: 20263 - protein, 9 aa, synthetic construct
GGKGNDIMA

SEQ ID NO: 20264 - protein, 9 aa, synthetic construct
GGKGNDLIV

SEQ ID NO: 20265 - protein, 9 aa, synthetic construct
GGKGNDLLW

SEQ ID NO: 20266 - protein, 9 aa, synthetic construct
GGKGNDRLH

SEQ ID NO: 20267 - protein, 9 aa, synthetic construct
GGKGNDLVD

SEQ ID NO: 20268 - protein, 9 aa, synthetic construct
GGKGNDRIH

SEQ ID NO: 20269 - protein, 9 aa, synthetic construct
GGKGNDRIF

SEQ ID NO: 20270 - protein, 9 aa, synthetic construct
GGDGNDQIE

SEQ ID NO: 20271 - protein, 9 aa, synthetic construct
GGKGNDQVW

SEQ ID NO: 20272 - protein, 9 aa, synthetic construct
GGDGNDQII

SEQ ID NO: 20273 - protein, 9 aa, synthetic construct
GGDGNDQIK

SEQ ID NO: 20274 - protein, 9 aa, synthetic construct
GGDGNDQIN

SEQ ID NO: 20275 - protein, 9 aa, synthetic construct
GGDGNDQIQ

SEQ ID NO: 20276 - protein, 9 aa, synthetic construct
GGDGNDQIS

SEQ ID NO: 20277 - protein, 9 aa, synthetic construct
GGKGNDQLD

SEQ ID NO: 20278 - protein, 9 aa, synthetic construct
GGEGADWIL

SEQ ID NO: 20279 - protein, 9 aa, synthetic construct
GGKGNDQIL

SEQ ID NO: 20280 - protein, 9 aa, synthetic construct
GGKGNDNLQ

SEQ ID NO: 20281 - protein, 9 aa, synthetic construct
GGKGNDMLT

SEQ ID NO: 20282 - protein, 9 aa, synthetic construct
GGKGNDLYV

SEQ ID NO: 20283 - protein, 9 aa, synthetic construct
GGDGEDTAV

SEQ ID NO: 20284 - protein, 9 aa, synthetic construct
GGKGNDILH

SEQ ID NO: 20285 - protein, 9 aa, synthetic construct
GGKGNDILC

SEQ ID NO: 20286 - protein, 9 aa, synthetic construct
GGGGNDNVK

SEQ ID NO: 20287 - protein, 9 aa, synthetic construct
GGKGNDAVR

SEQ ID NO: 20288 - protein, 9 aa, synthetic construct
GGKGNDALT

SEQ ID NO: 20289 - protein, 9 aa, synthetic construct
GGKGNDALF

SEQ ID NO: 20290 - protein, 9 aa, synthetic construct
GGKGMDVLT

SEQ ID NO: 20291 - protein, 9 aa, synthetic construct
GGKGMDRFY

SEQ ID NO: 20292 - protein, 9 aa, synthetic construct
GGKGMDQIT

SEQ ID NO: 20293 - protein, 9 aa, synthetic construct
GGKGLDYLY

SEQ ID NO: 20294 - protein, 9 aa, synthetic construct
GGKGLDVID

SEQ ID NO: 20295 - protein, 9 aa, synthetic construct
GGKGLDTLF

SEQ ID NO: 20296 - protein, 9 aa, synthetic construct
GGKGLDKLI

SEQ ID NO: 20297 - protein, 9 aa, synthetic construct
GGDGNDRMI

SEQ ID NO: 20298 - protein, 9 aa, synthetic construct
GGDGNDRMK

SEQ ID NO: 20299 - protein, 9 aa, synthetic construct
GGGGNDQID

SEQ ID NO: 20300 - protein, 9 aa, synthetic construct
GGDGNDRMM

SEQ ID NO: 20301 - protein, 9 aa, synthetic construct
GGKGKDVML

SEQ ID NO: 20302 - protein, 9 aa, synthetic construct
GGGGNDQFF

SEQ ID NO: 20303 - protein, 9 aa, synthetic construct
GGKGNDDLY

SEQ ID NO: 20304 - protein, 9 aa, synthetic construct
GGDGNDRIK

SEQ ID NO: 20305 - protein, 9 aa, synthetic construct
GGKGNDFMR

SEQ ID NO: 20306 - protein, 9 aa, synthetic construct
GGDGNDQYY

SEQ ID NO: 20307 - protein, 9 aa, synthetic construct
GGKGNDHLY

SEQ ID NO: 20308 - protein, 9 aa, synthetic construct
GGKGNDHLW

SEQ ID NO: 20309 - protein, 9 aa, synthetic construct
GGDGNDRAS

SEQ ID NO: 20310 - protein, 9 aa, synthetic construct
GGKGNDHLE

SEQ ID NO: 20311 - protein, 9 aa, synthetic construct
GGDGNDRAW

SEQ ID NO: 20312 - protein, 9 aa, synthetic construct
GGKGNDFMG

SEQ ID NO: 20313 - protein, 9 aa, synthetic construct
GGGGNDNYV

SEQ ID NO: 20314 - protein, 9 aa, synthetic construct
GGKGNDFLY

SEQ ID NO: 20315 - protein, 9 aa, synthetic construct
GGDGNDRFV

SEQ ID NO: 20316 - protein, 9 aa, synthetic construct
GGKGNDFLF

SEQ ID NO: 20317 - protein, 9 aa, synthetic construct
GGKGNDFLD

SEQ ID NO: 20318 - protein, 9 aa, synthetic construct
GGKGNDEVD

SEQ ID NO: 20319 - protein, 9 aa, synthetic construct
GGKGNDELN

SEQ ID NO: 20320 - protein, 9 aa, synthetic construct
GGKGNDRIQ

SEQ ID NO: 20321 - protein, 9 aa, synthetic construct
GGKGNDRLQ

SEQ ID NO: 20322 - protein, 9 aa, synthetic construct
GGKGKDVLQ

SEQ ID NO: 20323 - protein, 9 aa, synthetic construct
GGKGRDDLF

SEQ ID NO: 20324 - protein, 9 aa, synthetic construct
GGKGQDYID

SEQ ID NO: 20325 - protein, 9 aa, synthetic construct
GGGGNDMIT

SEQ ID NO: 20326 - protein, 9 aa, synthetic construct
GGDGNDLYY

SEQ ID NO: 20327 - protein, 9 aa, synthetic construct
GGGGNDMLA

SEQ ID NO: 20328 - protein, 9 aa, synthetic construct
GGKGQDTLT

SEQ ID NO: 20329 - protein, 9 aa, synthetic construct
GGKGQDTLS

SEQ ID NO: 20330 - protein, 9 aa, synthetic construct
GGDGNDMIN

SEQ ID NO: 20331 - protein, 9 aa, synthetic construct
GGKGQDSLS

SEQ ID NO: 20332 - protein, 9 aa, synthetic construct
GGKGQDLLQ

SEQ ID NO: 20333 - protein, 9 aa, synthetic construct
GGKGQDILT

SEQ ID NO: 20334 - protein, 9 aa, synthetic construct
GGGGNDMLI

SEQ ID NO: 20335 - protein, 9 aa, synthetic construct
GGKGQDALS

SEQ ID NO: 20336 - protein, 9 aa, synthetic construct
GGKGPDVLV

SEQ ID NO: 20337 - protein, 9 aa, synthetic construct
GGKGPDKLF

SEQ ID NO: 20338 - protein, 9 aa, synthetic construct
GGGGNDMLK

SEQ ID NO: 20339 - protein, 9 aa, synthetic construct
GGKGRDCLK

SEQ ID NO: 20340 - protein, 9 aa, synthetic construct
GGKGRDDLL

SEQ ID NO: 20341 - protein, 9 aa, synthetic construct
GGGGNDNLQ

SEQ ID NO: 20342 - protein, 9 aa, synthetic construct
GGDGNDLVQ

SEQ ID NO: 20343 - protein, 9 aa, synthetic construct
GGDGNDLMN

SEQ ID NO: 20344 - protein, 9 aa, synthetic construct
GGKGRDLIY

SEQ ID NO: 20345 - protein, 9 aa, synthetic construct
GGDGNDLMT

SEQ ID NO: 20346 - protein, 9 aa, synthetic construct
GGKGRDLIN

SEQ ID NO: 20347 - protein, 9 aa, synthetic construct
GGEGADYIW

SEQ ID NO: 20348 - protein, 9 aa, synthetic construct
GGKGRDKID

SEQ ID NO: 20349 - protein, 9 aa, synthetic construct
GGKGRDIVA

SEQ ID NO: 20350 - protein, 9 aa, synthetic construct
GGKGRDILS

SEQ ID NO: 20351 - protein, 9 aa, synthetic construct
GGKGRDILI

SEQ ID NO: 20352 - protein, 9 aa, synthetic construct
GGDGNDLVG

SEQ ID NO: 20353 - protein, 9 aa, synthetic construct
GGKGRDIFV

SEQ ID NO: 20354 - protein, 9 aa, synthetic construct
GGKGRDHLE

SEQ ID NO: 20355 - protein, 9 aa, synthetic construct
GGDGNDLVK

SEQ ID NO: 20356 - protein, 9 aa, synthetic construct
GGKGRDFLM

SEQ ID NO: 20357 - protein, 9 aa, synthetic construct
GGKGRDFLD

SEQ ID NO: 20358 - protein, 9 aa, synthetic construct
GGKGNDYLI

SEQ ID NO: 20359 - protein, 9 aa, synthetic construct
GGDGNDMMQ

SEQ ID NO: 20360 - protein, 9 aa, synthetic construct
GGEGADWVR

SEQ ID NO: 20361 - protein, 9 aa, synthetic construct
GGKGNDYFA

SEQ ID NO: 20362 - protein, 9 aa, synthetic construct
GGKGNDTIF

SEQ ID NO: 20363 - protein, 9 aa, synthetic construct
GGKGNDTIE

SEQ ID NO: 20364 - protein, 9 aa, synthetic construct
GGDGNDNLI

SEQ ID NO: 20365 - protein, 9 aa, synthetic construct
GGKGNDTFQ

SEQ ID NO: 20366 - protein, 9 aa, synthetic construct
GGDGNDNLW

SEQ ID NO: 20367 - protein, 9 aa, synthetic construct
GGKGNDSYL

SEQ ID NO: 20368 - protein, 9 aa, synthetic construct
GGEGADWLF

SEQ ID NO: 20369 - protein, 9 aa, synthetic construct
GGKGNDSML

SEQ ID NO: 20370 - protein, 9 aa, synthetic construct
GGKGNDSLL

SEQ ID NO: 20371 - protein, 9 aa, synthetic construct
GGKGNDSIT

SEQ ID NO: 20372 - protein, 9 aa, synthetic construct
GGKGNDSID

SEQ ID NO: 20373 - protein, 9 aa, synthetic construct
GGDGNDNVL

SEQ ID NO: 20374 - protein, 9 aa, synthetic construct
GGGGNDNLI

SEQ ID NO: 20375 - protein, 9 aa, synthetic construct
GGGGNDNLN

SEQ ID NO: 20376 - protein, 9 aa, synthetic construct
GGKGNDRLY

SEQ ID NO: 20377 - protein, 9 aa, synthetic construct
GGKGNDTIL

SEQ ID NO: 20378 - protein, 9 aa, synthetic construct
GGKGNDTIQ

SEQ ID NO: 20379 - protein, 9 aa, synthetic construct
GGDGNDNLH

SEQ ID NO: 20380 - protein, 9 aa, synthetic construct
GGEGADWLS

SEQ ID NO: 20381 - protein, 9 aa, synthetic construct
GGDGNDMVS

SEQ ID NO: 20382 - protein, 9 aa, synthetic construct
GGDGNDNFE

SEQ ID NO: 20383 - protein, 9 aa, synthetic construct
GGKGNDVYY

SEQ ID NO: 20384 - protein, 9 aa, synthetic construct
GGKGNDVLK

SEQ ID NO: 20385 - protein, 9 aa, synthetic construct
GGKGNDVIY

SEQ ID NO: 20386 - protein, 9 aa, synthetic construct
GGKGNDVIT

SEQ ID NO: 20387 - protein, 9 aa, synthetic construct
GGGGNDNAS

SEQ ID NO: 20388 - protein, 9 aa, synthetic construct
GGKGNDTIT

SEQ ID NO: 20389 - protein, 9 aa, synthetic construct
GGKGNDTYH

SEQ ID NO: 20390 - protein, 9 aa, synthetic construct
GGGGNDNID

SEQ ID NO: 20391 - protein, 9 aa, synthetic construct
GGKGNDTVS

SEQ ID NO: 20392 - protein, 9 aa, synthetic construct
GGKGNDTVL

SEQ ID NO: 20393 - protein, 9 aa, synthetic construct
GGKGNDTMG

SEQ ID NO: 20394 - protein, 9 aa, synthetic construct
GGDGNDNLG

SEQ ID NO: 20395 - protein, 9 aa, synthetic construct
GGDGNDRMS

SEQ ID NO: 20396 - protein, 9 aa, synthetic construct
GGKGKDVLL

SEQ ID NO: 20397 - protein, 9 aa, synthetic construct
GGLGDDILA

SEQ ID NO: 20398 - protein, 9 aa, synthetic construct
GGDGNDVFI

SEQ ID NO: 20399 - protein, 9 aa, synthetic construct
GGKGDDTVL

SEQ ID NO: 20400 - protein, 9 aa, synthetic construct
GGKGDDTVE

SEQ ID NO: 20401 - protein, 9 aa, synthetic construct
GGKGDDTLK

SEQ ID NO: 20402 - protein, 9 aa, synthetic construct
GGKGDDTIT

SEQ ID NO: 20403 - protein, 9 aa, synthetic construct
GGKGDDTIS

SEQ ID NO: 20404 - protein, 9 aa, synthetic construct
GGKGDDTIQ

SEQ ID NO: 20405 - protein, 9 aa, synthetic construct
GGKGDDTFY

SEQ ID NO: 20406 - protein, 9 aa, synthetic construct
GGKGDDTFV

SEQ ID NO: 20407 - protein, 9 aa, synthetic construct
GGKGDDTFN

SEQ ID NO: 20408 - protein, 9 aa, synthetic construct
GGKGDDTAY

SEQ ID NO: 20409 - protein, 9 aa, synthetic construct
GGKGDDSYA

SEQ ID NO: 20410 - protein, 9 aa, synthetic construct
GGKGDDSIT

SEQ ID NO: 20411 - protein, 9 aa, synthetic construct
GGKGDDSIL

SEQ ID NO: 20412 - protein, 9 aa, synthetic construct
GGKGDDSIA

SEQ ID NO: 20413 - protein, 9 aa, synthetic construct
GGKGDDRYV

SEQ ID NO: 20414 - protein, 9 aa, synthetic construct
GGDGNDVFQ

SEQ ID NO: 20415 - protein, 9 aa, synthetic construct
GGKGDDVFV

SEQ ID NO: 20416 - protein, 9 aa, synthetic construct
GGKGEDTLE

SEQ ID NO: 20417 - protein, 9 aa, synthetic construct
GGDGNDVAN

SEQ ID NO: 20418 - protein, 9 aa, synthetic construct
GGKGEDRVS

SEQ ID NO: 20419 - protein, 9 aa, synthetic construct
GGKGEDIFL

SEQ ID NO: 20420 - protein, 9 aa, synthetic construct
GGKGDDYLN

SEQ ID NO: 20421 - protein, 9 aa, synthetic construct
GGGGNDRII

SEQ ID NO: 20422 - protein, 9 aa, synthetic construct
GGKGDDYIY

SEQ ID NO: 20423 - protein, 9 aa, synthetic construct
GGKGDDYIV

SEQ ID NO: 20424 - protein, 9 aa, synthetic construct
GGKGDDYIS

SEQ ID NO: 20425 - protein, 9 aa, synthetic construct
GGDGNDTYC

SEQ ID NO: 20426 - protein, 9 aa, synthetic construct
GGKGDDWLR

SEQ ID NO: 20427 - protein, 9 aa, synthetic construct
GGKGDDVYK

SEQ ID NO: 20428 - protein, 9 aa, synthetic construct
GGKGDDVYI

SEQ ID NO: 20429 - protein, 9 aa, synthetic construct
GGKGDDVVS

SEQ ID NO: 20430 - protein, 9 aa, synthetic construct
GGKGDDVVM

SEQ ID NO: 20431 - protein, 9 aa, synthetic construct
GGKGDDVVE

SEQ ID NO: 20432 - protein, 9 aa, synthetic construct
GGEGADVLA

SEQ ID NO: 20433 - protein, 9 aa, synthetic construct
GGKGDDRME

SEQ ID NO: 20434 - protein, 9 aa, synthetic construct
GGKGDDRLV

SEQ ID NO: 20435 - protein, 9 aa, synthetic construct
GGKGDDRLN

SEQ ID NO: 20436 - protein, 9 aa, synthetic construct
GGKGDDRLI

SEQ ID NO: 20437 - protein, 9 aa, synthetic construct
GGKGDDKLD

SEQ ID NO: 20438 - protein, 9 aa, synthetic construct
GGDGNDVVT

SEQ ID NO: 20439 - protein, 9 aa, synthetic construct
GGGGNDRLK

SEQ ID NO: 20440 - protein, 9 aa, synthetic construct
GGKGDDKIE

SEQ ID NO: 20441 - protein, 9 aa, synthetic construct
GGKGDDKAQ

SEQ ID NO: 20442 - protein, 9 aa, synthetic construct
GGDGNDVVY

SEQ ID NO: 20443 - protein, 9 aa, synthetic construct
GGGGNDRLM

SEQ ID NO: 20444 - protein, 9 aa, synthetic construct
GGDGNDVYH

SEQ ID NO: 20445 - protein, 9 aa, synthetic construct
GGKGDDILM

SEQ ID NO: 20446 - protein, 9 aa, synthetic construct
GGKGDDILK

SEQ ID NO: 20447 - protein, 9 aa, synthetic construct
GGKGDDIIT

SEQ ID NO: 20448 - protein, 9 aa, synthetic construct
GGKGDDIIN

SEQ ID NO: 20449 - protein, 9 aa, synthetic construct
GGKGDDIIH

SEQ ID NO: 20450 - protein, 9 aa, synthetic construct
GGKGDDIIG

SEQ ID NO: 20451 - protein, 9 aa, synthetic construct
GGDGNDWFQ

SEQ ID NO: 20452 - protein, 9 aa, synthetic construct
GGDGNDVVL

SEQ ID NO: 20453 - protein, 9 aa, synthetic construct
GGKGDDKVY

SEQ ID NO: 20454 - protein, 9 aa, synthetic construct
GGKGDDLAI

SEQ ID NO: 20455 - protein, 9 aa, synthetic construct
GGKGDDMLR

SEQ ID NO: 20456 - protein, 9 aa, synthetic construct
GGKGDDRLA

SEQ ID NO: 20457 - protein, 9 aa, synthetic construct
GGKGDDQLN

SEQ ID NO: 20458 - protein, 9 aa, synthetic construct
GGKGDDQLI

SEQ ID NO: 20459 - protein, 9 aa, synthetic construct
GGKGDDNLQ

SEQ ID NO: 20460 - protein, 9 aa, synthetic construct
GGKGDDNLN

SEQ ID NO: 20461 - protein, 9 aa, synthetic construct
GGDGNDVMG

SEQ ID NO: 20462 - protein, 9 aa, synthetic construct
GGDGNDVML

SEQ ID NO: 20463 - protein, 9 aa, synthetic construct
GGDGNDVVI

SEQ ID NO: 20464 - protein, 9 aa, synthetic construct
GGKGDDLYL

SEQ ID NO: 20465 - protein, 9 aa, synthetic construct
GGDGNDVMR

SEQ ID NO: 20466 - protein, 9 aa, synthetic construct
GGKGDDLVE

SEQ ID NO: 20467 - protein, 9 aa, synthetic construct
GGKGDDLIV

SEQ ID NO: 20468 - protein, 9 aa, synthetic construct
GGKGDDLIS

SEQ ID NO: 20469 - protein, 9 aa, synthetic construct
GGDGNDVVG

SEQ ID NO: 20470 - protein, 9 aa, synthetic construct
GGEGADVLE

SEQ ID NO: 20471 - protein, 9 aa, synthetic construct
GGKGEDTLS

SEQ ID NO: 20472 - protein, 9 aa, synthetic construct
GGKGKDVIK

SEQ ID NO: 20473 - protein, 9 aa, synthetic construct
GGKGKDKLT

SEQ ID NO: 20474 - protein, 9 aa, synthetic construct
GGKGKDHLD

SEQ ID NO: 20475 - protein, 9 aa, synthetic construct
GGKGKDELF

SEQ ID NO: 20476 - protein, 9 aa, synthetic construct
GGKGKDAVY

SEQ ID NO: 20477 - protein, 9 aa, synthetic construct
GGDGNDSLQ

SEQ ID NO: 20478 - protein, 9 aa, synthetic construct
GGKGIDTFR

SEQ ID NO: 20479 - protein, 9 aa, synthetic construct
GGDGNDSME

SEQ ID NO: 20480 - protein, 9 aa, synthetic construct
GGKGIDRMF

SEQ ID NO: 20481 - protein, 9 aa, synthetic construct
GGKGIDIMQ

SEQ ID NO: 20482 - protein, 9 aa, synthetic construct
GGKGIDILT

SEQ ID NO: 20483 - protein, 9 aa, synthetic construct
GGDGNDSMW

SEQ ID NO: 20484 - protein, 9 aa, synthetic construct
GGKGHDYLG

SEQ ID NO: 20485 - protein, 9 aa, synthetic construct
GGKGHDYLD

SEQ ID NO: 20486 - protein, 9 aa, synthetic construct
GGKGHDVLN

SEQ ID NO: 20487 - protein, 9 aa, synthetic construct
GGDGNDSVI

SEQ ID NO: 20488 - protein, 9 aa, synthetic construct
GGKGHDVIY

SEQ ID NO: 20489 - protein, 9 aa, synthetic construct
GGKGKDILS

SEQ ID NO: 20490 - protein, 9 aa, synthetic construct
GGDGNDSIM

SEQ ID NO: 20491 - protein, 9 aa, synthetic construct
GGDGNDTMH

SEQ ID NO: 20492 - protein, 9 aa, synthetic construct
GGKGKDLLS

SEQ ID NO: 20493 - protein, 9 aa, synthetic construct
GGDGNDRVI

SEQ ID NO: 20494 - protein, 9 aa, synthetic construct
GGDGNDRVN

SEQ ID NO: 20495 - protein, 9 aa, synthetic construct
GGKGKDTLQ

SEQ ID NO: 20496 - protein, 9 aa, synthetic construct
GGKGKDTIN

SEQ ID NO: 20497 - protein, 9 aa, synthetic construct
GGGGNDQIV

SEQ ID NO: 20498 - protein, 9 aa, synthetic construct
GGKGKDTFA

SEQ ID NO: 20499 - protein, 9 aa, synthetic construct
GGGGNDQIY

SEQ ID NO: 20500 - protein, 9 aa, synthetic construct
GGKGKDSII

SEQ ID NO: 20501 - protein, 9 aa, synthetic construct
GGKGKDRLV

SEQ ID NO: 20502 - protein, 9 aa, synthetic construct
GGKGKDRLT

SEQ ID NO: 20503 - protein, 9 aa, synthetic construct
GGKGKDRLF

SEQ ID NO: 20504 - protein, 9 aa, synthetic construct
GGKGKDQLE

SEQ ID NO: 20505 - protein, 9 aa, synthetic construct
GGGGNDQLN

SEQ ID NO: 20506 - protein, 9 aa, synthetic construct
GGKGKDNYG

SEQ ID NO: 20507 - protein, 9 aa, synthetic construct
GGGGNDQLQ

SEQ ID NO: 20508 - protein, 9 aa, synthetic construct
GGKGHDVID

SEQ ID NO: 20509 - protein, 9 aa, synthetic construct
GGDGNDSVT

SEQ ID NO: 20510 - protein, 9 aa, synthetic construct
GGDGNDSYF

SEQ ID NO: 20511 - protein, 9 aa, synthetic construct
GGDGNDSYH

SEQ ID NO: 20512 - protein, 9 aa, synthetic construct
GGGGNDRFS

SEQ ID NO: 20513 - protein, 9 aa, synthetic construct
GGKGGDVFI

SEQ ID NO: 20514 - protein, 9 aa, synthetic construct
GGDGNDTFS

SEQ ID NO: 20515 - protein, 9 aa, synthetic construct
GGDGNDTFT

SEQ ID NO: 20516 - protein, 9 aa, synthetic construct
GGKGGDTLD

SEQ ID NO: 20517 - protein, 9 aa, synthetic construct
GGKGGDTFI

SEQ ID NO: 20518 - protein, 9 aa, synthetic construct
GGKGGDSLT

SEQ ID NO: 20519 - protein, 9 aa, synthetic construct
GGKGGDRLR

SEQ ID NO: 20520 - protein, 9 aa, synthetic construct
GGKGGDQLD

SEQ ID NO: 20521 - protein, 9 aa, synthetic construct
GGKGGDHLD

SEQ ID NO: 20522 - protein, 9 aa, synthetic construct
GGKGGDALF

SEQ ID NO: 20523 - protein, 9 aa, synthetic construct
GGKGFDQIA

SEQ ID NO: 20524 - protein, 9 aa, synthetic construct
GGKGFDDIK

SEQ ID NO: 20525 - protein, 9 aa, synthetic construct
GGKGEDVLS

SEQ ID NO: 20526 - protein, 9 aa, synthetic construct
GGKGEDVIL

SEQ ID NO: 20527 - protein, 9 aa, synthetic construct
GGGGNDRFI

SEQ ID NO: 20528 - protein, 9 aa, synthetic construct
GGKGHDHYI

SEQ ID NO: 20529 - protein, 9 aa, synthetic construct
GGKGHDILN

SEQ ID NO: 20530 - protein, 9 aa, synthetic construct
GGDGNDSYV

SEQ ID NO: 20531 - protein, 9 aa, synthetic construct
GGKGHDSYI

SEQ ID NO: 20532 - protein, 9 aa, synthetic construct
GGKGHDSLV

SEQ ID NO: 20533 - protein, 9 aa, synthetic construct
GGDGNDSYI

SEQ ID NO: 20534 - protein, 9 aa, synthetic construct
GGKGHDSLD

SEQ ID NO: 20535 - protein, 9 aa, synthetic construct
GGDGNDSYT

SEQ ID NO: 20536 - protein, 9 aa, synthetic construct
GGKGHDSIE

SEQ ID NO: 20537 - protein, 9 aa, synthetic construct
GGKGHDRLH

SEQ ID NO: 20538 - protein, 9 aa, synthetic construct
GGKGHDIMR

SEQ ID NO: 20539 - protein, 9 aa, synthetic construct
GGKGHDRLA

SEQ ID NO: 20540 - protein, 9 aa, synthetic construct
GGKGHDLLL

SEQ ID NO: 20541 - protein, 9 aa, synthetic construct
GGDGNDTAI

SEQ ID NO: 20542 - protein, 9 aa, synthetic construct
GGKGHDLII

SEQ ID NO: 20543 - protein, 9 aa, synthetic construct
GGDGNDTAQ

SEQ ID NO: 20544 - protein, 9 aa, synthetic construct
GGDGNDTAR

SEQ ID NO: 20545 - protein, 9 aa, synthetic construct
GGKGRDMLT

SEQ ID NO: 20546 - protein, 9 aa, synthetic construct
GGDGNDLML

SEQ ID NO: 20547 - protein, 9 aa, synthetic construct
GGKGRDMLW

SEQ ID NO: 20548 - protein, 9 aa, synthetic construct
GGLGADSIL

SEQ ID NO: 20549 - protein, 9 aa, synthetic construct
GGLGADSIE

SEQ ID NO: 20550 - protein, 9 aa, synthetic construct
GGLGADSID

SEQ ID NO: 20551 - protein, 9 aa, synthetic construct
GGDGNDEME

SEQ ID NO: 20552 - protein, 9 aa, synthetic construct
GGLGADSFL

SEQ ID NO: 20553 - protein, 9 aa, synthetic construct
GGLGADSFI

SEQ ID NO: 20554 - protein, 9 aa, synthetic construct
GGLGADSAF

SEQ ID NO: 20555 - protein, 9 aa, synthetic construct
GGLGADRMY

SEQ ID NO: 20556 - protein, 9 aa, synthetic construct
GGLGADRMT

SEQ ID NO: 20557 - protein, 9 aa, synthetic construct
GGLGADRMD

SEQ ID NO: 20558 - protein, 9 aa, synthetic construct
GGLGADRLM

SEQ ID NO: 20559 - protein, 9 aa, synthetic construct
GGDGNDEMY

SEQ ID NO: 20560 - protein, 9 aa, synthetic construct
GGGGNDKFY

SEQ ID NO: 20561 - protein, 9 aa, synthetic construct
GGLGADRIL

SEQ ID NO: 20562 - protein, 9 aa, synthetic construct
GGLGADRII

SEQ ID NO: 20563 - protein, 9 aa, synthetic construct
GGLGADRIF

SEQ ID NO: 20564 - protein, 9 aa, synthetic construct
GGLGADSII

SEQ ID NO: 20565 - protein, 9 aa, synthetic construct
GGLGADSLW

SEQ ID NO: 20566 - protein, 9 aa, synthetic construct
GGLGADVIK

SEQ ID NO: 20567 - protein, 9 aa, synthetic construct
GGLGADSML

SEQ ID NO: 20568 - protein, 9 aa, synthetic construct
GGLGADTYY

SEQ ID NO: 20569 - protein, 9 aa, synthetic construct
GGLGADTYV

SEQ ID NO: 20570 - protein, 9 aa, synthetic construct
GGLGADTYK

SEQ ID NO: 20571 - protein, 9 aa, synthetic construct
GGLGADTYF

SEQ ID NO: 20572 - protein, 9 aa, synthetic construct
GGLGADTYA

SEQ ID NO: 20573 - protein, 9 aa, synthetic construct
GGLGADTMM

SEQ ID NO: 20574 - protein, 9 aa, synthetic construct
GGLGADTMK

SEQ ID NO: 20575 - protein, 9 aa, synthetic construct
GGDGNDEII

SEQ ID NO: 20576 - protein, 9 aa, synthetic construct
GGLGADTMF

SEQ ID NO: 20577 - protein, 9 aa, synthetic construct
GGLGADTLG

SEQ ID NO: 20578 - protein, 9 aa, synthetic construct
GGLGADTIV

SEQ ID NO: 20579 - protein, 9 aa, synthetic construct
GGLGADTFS

SEQ ID NO: 20580 - protein, 9 aa, synthetic construct
GGLGADTFL

SEQ ID NO: 20581 - protein, 9 aa, synthetic construct
GGLGADTFF

SEQ ID NO: 20582 - protein, 9 aa, synthetic construct
GGDGNDELN

SEQ ID NO: 20583 - protein, 9 aa, synthetic construct
GGLGADRFW

SEQ ID NO: 20584 - protein, 9 aa, synthetic construct
GGLGADRFL

SEQ ID NO: 20585 - protein, 9 aa, synthetic construct
GGDGNDFAQ

SEQ ID NO: 20586 - protein, 9 aa, synthetic construct
GGDGNDFAV

SEQ ID NO: 20587 - protein, 9 aa, synthetic construct
GGLGADMLD

SEQ ID NO: 20588 - protein, 9 aa, synthetic construct
GGLGADMLA

SEQ ID NO: 20589 - protein, 9 aa, synthetic construct
GGLGADLVI

SEQ ID NO: 20590 - protein, 9 aa, synthetic construct
GGLGADLMN

SEQ ID NO: 20591 - protein, 9 aa, synthetic construct
GGLGADLMI

SEQ ID NO: 20592 - protein, 9 aa, synthetic construct
GGLGADLMF

SEQ ID NO: 20593 - protein, 9 aa, synthetic construct
GGDGNDFVA

SEQ ID NO: 20594 - protein, 9 aa, synthetic construct
GGLGADLLY

SEQ ID NO: 20595 - protein, 9 aa, synthetic construct
GGLGADLLQ

SEQ ID NO: 20596 - protein, 9 aa, synthetic construct
GGLGADLLL

SEQ ID NO: 20597 - protein, 9 aa, synthetic construct
GGLGADLLK

SEQ ID NO: 20598 - protein, 9 aa, synthetic construct
GGLGADLLE

SEQ ID NO: 20599 - protein, 9 aa, synthetic construct
GGLGADLLA

SEQ ID NO: 20600 - protein, 9 aa, synthetic construct
GGDGNDFVD

SEQ ID NO: 20601 - protein, 9 aa, synthetic construct
GGLGADLIL

SEQ ID NO: 20602 - protein, 9 aa, synthetic construct
GGDGNDFLT

SEQ ID NO: 20603 - protein, 9 aa, synthetic construct
GGLGADMLL

SEQ ID NO: 20604 - protein, 9 aa, synthetic construct
GGLGADNIA

SEQ ID NO: 20605 - protein, 9 aa, synthetic construct
GGLGADQLV

SEQ ID NO: 20606 - protein, 9 aa, synthetic construct
GGGGNDKIT

SEQ ID NO: 20607 - protein, 9 aa, synthetic construct
GGLGADQMT

SEQ ID NO: 20608 - protein, 9 aa, synthetic construct
GGEGDDAFD

SEQ ID NO: 20609 - protein, 9 aa, synthetic construct
GGLGADQMI

SEQ ID NO: 20610 - protein, 9 aa, synthetic construct
GGLGADQMD

SEQ ID NO: 20611 - protein, 9 aa, synthetic construct
GGDGNDFIF

SEQ ID NO: 20612 - protein, 9 aa, synthetic construct
GGDGNDFIL

SEQ ID NO: 20613 - protein, 9 aa, synthetic construct
GGGGNDKLD

SEQ ID NO: 20614 - protein, 9 aa, synthetic construct
GGDGNDFIQ

SEQ ID NO: 20615 - protein, 9 aa, synthetic construct
GGDGNDFIR

SEQ ID NO: 20616 - protein, 9 aa, synthetic construct
GGLGADQLE

SEQ ID NO: 20617 - protein, 9 aa, synthetic construct
GGLGADQIW

SEQ ID NO: 20618 - protein, 9 aa, synthetic construct
GGGGNDKLA

SEQ ID NO: 20619 - protein, 9 aa, synthetic construct
GGLGADNLQ

SEQ ID NO: 20620 - protein, 9 aa, synthetic construct
GGLGADVFL

SEQ ID NO: 20621 - protein, 9 aa, synthetic construct
GGLGADVIS

SEQ ID NO: 20622 - protein, 9 aa, synthetic construct
GGKGRDRID

SEQ ID NO: 20623 - protein, 9 aa, synthetic construct
GGDGNDAFV

SEQ ID NO: 20624 - protein, 9 aa, synthetic construct
GGLGDDFYI

SEQ ID NO: 20625 - protein, 9 aa, synthetic construct
GGDGNDAIG

SEQ ID NO: 20626 - protein, 9 aa, synthetic construct
GGGGNDIIF

SEQ ID NO: 20627 - protein, 9 aa, synthetic construct
GGLGDDFLY

SEQ ID NO: 20628 - protein, 9 aa, synthetic construct
GGLGDDFLQ

SEQ ID NO: 20629 - protein, 9 aa, synthetic construct
GGLGDDFLK

SEQ ID NO: 20630 - protein, 9 aa, synthetic construct
GGLGDDFLI

SEQ ID NO: 20631 - protein, 9 aa, synthetic construct
GGLGDDFLH

SEQ ID NO: 20632 - protein, 9 aa, synthetic construct
GGLGDDEYV

SEQ ID NO: 20633 - protein, 9 aa, synthetic construct
GGLGDDEVY

SEQ ID NO: 20634 - protein, 9 aa, synthetic construct
GGLGDDEMQ

SEQ ID NO: 20635 - protein, 9 aa, synthetic construct
GGLGDDEMF

SEQ ID NO: 20636 - protein, 9 aa, synthetic construct
GGDGNDALE

SEQ ID NO: 20637 - protein, 9 aa, synthetic construct
GGDGNDALG

SEQ ID NO: 20638 - protein, 9 aa, synthetic construct
GGDGNDALM

SEQ ID NO: 20639 - protein, 9 aa, synthetic construct
GGDGNDAIF

SEQ ID NO: 20640 - protein, 9 aa, synthetic construct
GGLGDDGIV

SEQ ID NO: 20641 - protein, 9 aa, synthetic construct
GGLGADVLG

SEQ ID NO: 20642 - protein, 9 aa, synthetic construct
GGGGNDIIA

SEQ ID NO: 20643 - protein, 9 aa, synthetic construct
GGLGDDIIY

SEQ ID NO: 20644 - protein, 9 aa, synthetic construct
GGDGMDTLV

SEQ ID NO: 20645 - protein, 9 aa, synthetic construct
GGLGDDIII

SEQ ID NO: 20646 - protein, 9 aa, synthetic construct
GGLGDDIIA

SEQ ID NO: 20647 - protein, 9 aa, synthetic construct
GGLGDDIFY

SEQ ID NO: 20648 - protein, 9 aa, synthetic construct
GGGGNDIFC

SEQ ID NO: 20649 - protein, 9 aa, synthetic construct
GGLGDDHLY

SEQ ID NO: 20650 - protein, 9 aa, synthetic construct
GGLGDDHLV

SEQ ID NO: 20651 - protein, 9 aa, synthetic construct
GGLGDDHLF

SEQ ID NO: 20652 - protein, 9 aa, synthetic construct
GGLGDDHIW

SEQ ID NO: 20653 - protein, 9 aa, synthetic construct
GGGGNDIFL

SEQ ID NO: 20654 - protein, 9 aa, synthetic construct
GGLGDDHIF

SEQ ID NO: 20655 - protein, 9 aa, synthetic construct
GGLGDDGYM

SEQ ID NO: 20656 - protein, 9 aa, synthetic construct
GGLGDDGVE

SEQ ID NO: 20657 - protein, 9 aa, synthetic construct
GGDGMDYLS

SEQ ID NO: 20658 - protein, 9 aa, synthetic construct
GGLGDDEIY

SEQ ID NO: 20659 - protein, 9 aa, synthetic construct
GGLGDDEIR

SEQ ID NO: 20660 - protein, 9 aa, synthetic construct
GGLGDDEIN

SEQ ID NO: 20661 - protein, 9 aa, synthetic construct
GGEGDDAMT

SEQ ID NO: 20662 - protein, 9 aa, synthetic construct
GGLGADYLN

SEQ ID NO: 20663 - protein, 9 aa, synthetic construct
GGLGADYLD

SEQ ID NO: 20664 - protein, 9 aa, synthetic construct
GGLGADYIQ

SEQ ID NO: 20665 - protein, 9 aa, synthetic construct
GGDGNDDLA

SEQ ID NO: 20666 - protein, 9 aa, synthetic construct
GGLGADYID

SEQ ID NO: 20667 - protein, 9 aa, synthetic construct
GGLGADWMI

SEQ ID NO: 20668 - protein, 9 aa, synthetic construct
GGDGNDDLM

SEQ ID NO: 20669 - protein, 9 aa, synthetic construct
GGLGADWLL

SEQ ID NO: 20670 - protein, 9 aa, synthetic construct
GGDGNDDLV

SEQ ID NO: 20671 - protein, 9 aa, synthetic construct
GGLGADVVS

SEQ ID NO: 20672 - protein, 9 aa, synthetic construct
GGDGNDDLW

SEQ ID NO: 20673 - protein, 9 aa, synthetic construct
GGLGADVMR

SEQ ID NO: 20674 - protein, 9 aa, synthetic construct
GGLGADVMK

SEQ ID NO: 20675 - protein, 9 aa, synthetic construct
GGDGNDDMI

SEQ ID NO: 20676 - protein, 9 aa, synthetic construct
GGDGNDDMV

SEQ ID NO: 20677 - protein, 9 aa, synthetic construct
GGDGNDDIY

SEQ ID NO: 20678 - protein, 9 aa, synthetic construct
GGLGADYMA

SEQ ID NO: 20679 - protein, 9 aa, synthetic construct
GGDGNDDIM

SEQ ID NO: 20680 - protein, 9 aa, synthetic construct
GGGGNDIIT

SEQ ID NO: 20681 - protein, 9 aa, synthetic construct
GGLGDDDMD

SEQ ID NO: 20682 - protein, 9 aa, synthetic construct
GGGGNDIIR

SEQ ID NO: 20683 - protein, 9 aa, synthetic construct
GGLGDDDLR

SEQ ID NO: 20684 - protein, 9 aa, synthetic construct
GGDGNDAML

SEQ ID NO: 20685 - protein, 9 aa, synthetic construct
GGLGDDDLH

SEQ ID NO: 20686 - protein, 9 aa, synthetic construct
GGLGDDDLA

SEQ ID NO: 20687 - protein, 9 aa, synthetic construct
GGLGDDDID

SEQ ID NO: 20688 - protein, 9 aa, synthetic construct
GGDGNDDII

SEQ ID NO: 20689 - protein, 9 aa, synthetic construct
GGDGNDAVY

SEQ ID NO: 20690 - protein, 9 aa, synthetic construct
GGDGNDAYA

SEQ ID NO: 20691 - protein, 9 aa, synthetic construct
GGLGDDALY

SEQ ID NO: 20692 - protein, 9 aa, synthetic construct
GGLGDDALW

SEQ ID NO: 20693 - protein, 9 aa, synthetic construct
GGLGDDALS

SEQ ID NO: 20694 - protein, 9 aa, synthetic construct
GGDGNDCLF

SEQ ID NO: 20695 - protein, 9 aa, synthetic construct
GGDGNDFVF

SEQ ID NO: 20696 - protein, 9 aa, synthetic construct
GGLGADLIF

SEQ ID NO: 20697 - protein, 9 aa, synthetic construct
GGLGADLID

SEQ ID NO: 20698 - protein, 9 aa, synthetic construct
GGKGSDTIS

SEQ ID NO: 20699 - protein, 9 aa, synthetic construct
GGKGSDTFH

SEQ ID NO: 20700 - protein, 9 aa, synthetic construct
GGKGSDTAH

SEQ ID NO: 20701 - protein, 9 aa, synthetic construct
GGKGSDSMA

SEQ ID NO: 20702 - protein, 9 aa, synthetic construct
GGDGNDKIW

SEQ ID NO: 20703 - protein, 9 aa, synthetic construct
GGGGNDLMQ

SEQ ID NO: 20704 - protein, 9 aa, synthetic construct
GGKGSDRLD

SEQ ID NO: 20705 - protein, 9 aa, synthetic construct
GGKGSDRFY

SEQ ID NO: 20706 - protein, 9 aa, synthetic construct
GGKGSDQLD

SEQ ID NO: 20707 - protein, 9 aa, synthetic construct
GGKGSDMLT

SEQ ID NO: 20708 - protein, 9 aa, synthetic construct
GGKGSDMLF

SEQ ID NO: 20709 - protein, 9 aa, synthetic construct
GGKGSDLYQ

SEQ ID NO: 20710 - protein, 9 aa, synthetic construct
GGEGADYLN

SEQ ID NO: 20711 - protein, 9 aa, synthetic construct
GGKGSDLLS

SEQ ID NO: 20712 - protein, 9 aa, synthetic construct
GGKGSDLLI

SEQ ID NO: 20713 - protein, 9 aa, synthetic construct
GGKGSDLLA

SEQ ID NO: 20714 - protein, 9 aa, synthetic construct
GGEGADYMS

SEQ ID NO: 20715 - protein, 9 aa, synthetic construct
GGDGNDKFY

SEQ ID NO: 20716 - protein, 9 aa, synthetic construct
GGLGADKMT

SEQ ID NO: 20717 - protein, 9 aa, synthetic construct
GGKGSDTLN

SEQ ID NO: 20718 - protein, 9 aa, synthetic construct
GGKGTDTLL

SEQ ID NO: 20719 - protein, 9 aa, synthetic construct
GGKGTDSLI

SEQ ID NO: 20720 - protein, 9 aa, synthetic construct
GGKGTDMLK

SEQ ID NO: 20721 - protein, 9 aa, synthetic construct
GGKGTDIVT

SEQ ID NO: 20722 - protein, 9 aa, synthetic construct
GGDGNDIMA

SEQ ID NO: 20723 - protein, 9 aa, synthetic construct
GGDGNDIMD

SEQ ID NO: 20724 - protein, 9 aa, synthetic construct
GGKGSDWMK

SEQ ID NO: 20725 - protein, 9 aa, synthetic construct
GGKGSDVLQ

SEQ ID NO: 20726 - protein, 9 aa, synthetic construct
GGKGSDVLD

SEQ ID NO: 20727 - protein, 9 aa, synthetic construct
GGKGSDVLA

SEQ ID NO: 20728 - protein, 9 aa, synthetic construct
GGDGNDIVH

SEQ ID NO: 20729 - protein, 9 aa, synthetic construct
GGDGNDIVL

SEQ ID NO: 20730 - protein, 9 aa, synthetic construct
GGDGNDIYL

SEQ ID NO: 20731 - protein, 9 aa, synthetic construct
GGKGSDTMF

SEQ ID NO: 20732 - protein, 9 aa, synthetic construct
GGKGSDTLW

SEQ ID NO: 20733 - protein, 9 aa, synthetic construct
GGDGNDKVD

SEQ ID NO: 20734 - protein, 9 aa, synthetic construct
GGKGSDLAV

SEQ ID NO: 20735 - protein, 9 aa, synthetic construct
GGDGNDKVI

SEQ ID NO: 20736 - protein, 9 aa, synthetic construct
GGKGSDKLR

SEQ ID NO: 20737 - protein, 9 aa, synthetic construct
GGEGADYLI

SEQ ID NO: 20738 - protein, 9 aa, synthetic construct
GGEGADYLH

SEQ ID NO: 20739 - protein, 9 aa, synthetic construct
GGDGNDLIQ

SEQ ID NO: 20740 - protein, 9 aa, synthetic construct
GGKGRDVLY

SEQ ID NO: 20741 - protein, 9 aa, synthetic construct
GGKGRDVLL

SEQ ID NO: 20742 - protein, 9 aa, synthetic construct
GGKGRDTLS

SEQ ID NO: 20743 - protein, 9 aa, synthetic construct
GGKGRDTLQ

SEQ ID NO: 20744 - protein, 9 aa, synthetic construct
GGKGRDTLD

SEQ ID NO: 20745 - protein, 9 aa, synthetic construct
GGKGRDTAV

SEQ ID NO: 20746 - protein, 9 aa, synthetic construct
GGKGRDSLV

SEQ ID NO: 20747 - protein, 9 aa, synthetic construct
GGKGRDSLL

SEQ ID NO: 20748 - protein, 9 aa, synthetic construct
GGKGRDSIM

SEQ ID NO: 20749 - protein, 9 aa, synthetic construct
GGKGRDSIH

SEQ ID NO: 20750 - protein, 9 aa, synthetic construct
GGKGRDRLF

SEQ ID NO: 20751 - protein, 9 aa, synthetic construct
GGKGRDRLE

SEQ ID NO: 20752 - protein, 9 aa, synthetic construct
GGKGSDDLF

SEQ ID NO: 20753 - protein, 9 aa, synthetic construct
GGKGSDEFN

SEQ ID NO: 20754 - protein, 9 aa, synthetic construct
GGKGSDFLS

SEQ ID NO: 20755 - protein, 9 aa, synthetic construct
GGDGNDLAD

SEQ ID NO: 20756 - protein, 9 aa, synthetic construct
GGDGNDKVL

SEQ ID NO: 20757 - protein, 9 aa, synthetic construct
GGGGNDLVH

SEQ ID NO: 20758 - protein, 9 aa, synthetic construct
GGGGNDLVL

SEQ ID NO: 20759 - protein, 9 aa, synthetic construct
GGGGNDLVN

SEQ ID NO: 20760 - protein, 9 aa, synthetic construct
GGKGSDIYV

SEQ ID NO: 20761 - protein, 9 aa, synthetic construct
GGDGNDKYY

SEQ ID NO: 20762 - protein, 9 aa, synthetic construct
GGDGNDLAY

SEQ ID NO: 20763 - protein, 9 aa, synthetic construct
GGKGSDFLY

SEQ ID NO: 20764 - protein, 9 aa, synthetic construct
GGDGNDLFF

SEQ ID NO: 20765 - protein, 9 aa, synthetic construct
GGKGSDILN

SEQ ID NO: 20766 - protein, 9 aa, synthetic construct
GGKGSDILL

SEQ ID NO: 20767 - protein, 9 aa, synthetic construct
GGKGSDILI

SEQ ID NO: 20768 - protein, 9 aa, synthetic construct
GGDGNDLFT

SEQ ID NO: 20769 - protein, 9 aa, synthetic construct
GGKGSDGLA

SEQ ID NO: 20770 - protein, 9 aa, synthetic construct
GGKGTDTLV

SEQ ID NO: 20771 - protein, 9 aa, synthetic construct
GGKGVDFLS

SEQ ID NO: 20772 - protein, 9 aa, synthetic construct
GGDGNDIIM

SEQ ID NO: 20773 - protein, 9 aa, synthetic construct
GGLGADDLS

SEQ ID NO: 20774 - protein, 9 aa, synthetic construct
GGLGADGLN

SEQ ID NO: 20775 - protein, 9 aa, synthetic construct
GGLGADGLF

SEQ ID NO: 20776 - protein, 9 aa, synthetic construct
GGLGADGIA

SEQ ID NO: 20777 - protein, 9 aa, synthetic construct
GGLGADFMT

SEQ ID NO: 20778 - protein, 9 aa, synthetic construct
GGGGNDLFV

SEQ ID NO: 20779 - protein, 9 aa, synthetic construct
GGLGADFIY

SEQ ID NO: 20780 - protein, 9 aa, synthetic construct
GGGGNDLIA

SEQ ID NO: 20781 - protein, 9 aa, synthetic construct
GGLGADEMV

SEQ ID NO: 20782 - protein, 9 aa, synthetic construct
GGLGADELW

SEQ ID NO: 20783 - protein, 9 aa, synthetic construct
GGLGADELN

SEQ ID NO: 20784 - protein, 9 aa, synthetic construct
GGDGNDGVA

SEQ ID NO: 20785 - protein, 9 aa, synthetic construct
GGDGNDGVE

SEQ ID NO: 20786 - protein, 9 aa, synthetic construct
GGDGNDGVY

SEQ ID NO: 20787 - protein, 9 aa, synthetic construct
GGLGADEIF

SEQ ID NO: 20788 - protein, 9 aa, synthetic construct
GGGGNDLII

SEQ ID NO: 20789 - protein, 9 aa, synthetic construct
GGLGADHFA

SEQ ID NO: 20790 - protein, 9 aa, synthetic construct
GGEGCDTAG

SEQ ID NO: 20791 - protein, 9 aa, synthetic construct
GGLGADHLF

SEQ ID NO: 20792 - protein, 9 aa, synthetic construct
GGDGNDFVY

SEQ ID NO: 20793 - protein, 9 aa, synthetic construct
GGLGADKLV

SEQ ID NO: 20794 - protein, 9 aa, synthetic construct
GGDGNDFVS

SEQ ID NO: 20795 - protein, 9 aa, synthetic construct
GGLGADKLL

SEQ ID NO: 20796 - protein, 9 aa, synthetic construct
GGLGADKIY

SEQ ID NO: 20797 - protein, 9 aa, synthetic construct
GGLGADKIT

SEQ ID NO: 20798 - protein, 9 aa, synthetic construct
GGLGADKFV

SEQ ID NO: 20799 - protein, 9 aa, synthetic construct
GGEGCDTVR

SEQ ID NO: 20800 - protein, 9 aa, synthetic construct
GGGGNDLAT

SEQ ID NO: 20801 - protein, 9 aa, synthetic construct
GGLGADIVN

SEQ ID NO: 20802 - protein, 9 aa, synthetic construct
GGLGADIMK

SEQ ID NO: 20803 - protein, 9 aa, synthetic construct
GGDGNDGIS

SEQ ID NO: 20804 - protein, 9 aa, synthetic construct
GGDGNDGIT

SEQ ID NO: 20805 - protein, 9 aa, synthetic construct
GGLGADIII

SEQ ID NO: 20806 - protein, 9 aa, synthetic construct
GGLGADIID

SEQ ID NO: 20807 - protein, 9 aa, synthetic construct
GGDGNDHIF

SEQ ID NO: 20808 - protein, 9 aa, synthetic construct
GGDGNDHLA

SEQ ID NO: 20809 - protein, 9 aa, synthetic construct
GGKGVDKLS

SEQ ID NO: 20810 - protein, 9 aa, synthetic construct
GGLGADDFV

SEQ ID NO: 20811 - protein, 9 aa, synthetic construct
GGKGYDLFD

SEQ ID NO: 20812 - protein, 9 aa, synthetic construct
GGDGNDIAV

SEQ ID NO: 20813 - protein, 9 aa, synthetic construct
GGKGWDVLN

SEQ ID NO: 20814 - protein, 9 aa, synthetic construct
GGKGWDNMT

SEQ ID NO: 20815 - protein, 9 aa, synthetic construct
GGDGNDIFA

SEQ ID NO: 20816 - protein, 9 aa, synthetic construct
GGKGWDLLV

SEQ ID NO: 20817 - protein, 9 aa, synthetic construct
GGDGNDIFG

SEQ ID NO: 20818 - protein, 9 aa, synthetic construct
GGDGNDIFH

SEQ ID NO: 20819 - protein, 9 aa, synthetic construct
GGKGVDVMA

SEQ ID NO: 20820 - protein, 9 aa, synthetic construct
GGDGNDIFL

SEQ ID NO: 20821 - protein, 9 aa, synthetic construct
GGKGVDVLD

SEQ ID NO: 20822 - protein, 9 aa, synthetic construct
GGKGVDVAI

SEQ ID NO: 20823 - protein, 9 aa, synthetic construct
GGKGVDTLN

SEQ ID NO: 20824 - protein, 9 aa, synthetic construct
GGKGVDTAI

SEQ ID NO: 20825 - protein, 9 aa, synthetic construct
GGKGVDNID

SEQ ID NO: 20826 - protein, 9 aa, synthetic construct
GGKGYDLVY

SEQ ID NO: 20827 - protein, 9 aa, synthetic construct
GGDGNDIAL

SEQ ID NO: 20828 - protein, 9 aa, synthetic construct
GGDGNDIAI

SEQ ID NO: 20829 - protein, 9 aa, synthetic construct
GGDGNDHLL

SEQ ID NO: 20830 - protein, 9 aa, synthetic construct
GGLGADAMY

SEQ ID NO: 20831 - protein, 9 aa, synthetic construct
GGLGADAMV

SEQ ID NO: 20832 - protein, 9 aa, synthetic construct
GGLGADAMT

SEQ ID NO: 20833 - protein, 9 aa, synthetic construct
GGLGADAMR

SEQ ID NO: 20834 - protein, 9 aa, synthetic construct
GGLGADAML

SEQ ID NO: 20835 - protein, 9 aa, synthetic construct
GGLGADAMD

SEQ ID NO: 20836 - protein, 9 aa, synthetic construct
GGLGADALE

SEQ ID NO: 20837 - protein, 9 aa, synthetic construct
GGKGYDTLW

SEQ ID NO: 20838 - protein, 9 aa, synthetic construct
GGDGNDHLR

SEQ ID NO: 20839 - protein, 9 aa, synthetic construct
GGLGADAFV

SEQ ID NO: 20840 - protein, 9 aa, synthetic construct
GGDGNDHLW

SEQ ID NO: 20841 - protein, 9 aa, synthetic construct
GGLGADAFQ

SEQ ID NO: 20842 - protein, 9 aa, synthetic construct
GGKGYDTYY

SEQ ID NO: 20843 - protein, 9 aa, synthetic construct
GGKGYDTYV

SEQ ID NO: 20844 - protein, 9 aa, synthetic construct
GGMGADRLN

SEQ ID NO: 20845 - protein, 9 aa, synthetic construct
GGQGSDMLL

SEQ ID NO: 20846 - protein, 9 aa, synthetic construct
GGMGADRLT

SEQ ID NO: 20847 - protein, 9 aa, synthetic construct
GGFGDDYIA

SEQ ID NO: 20848 - protein, 9 aa, synthetic construct
GGSGVDFMR

SEQ ID NO: 20849 - protein, 9 aa, synthetic construct
GGAGIDVMT

SEQ ID NO: 20850 - protein, 9 aa, synthetic construct
GGAGIDVMV

SEQ ID NO: 20851 - protein, 9 aa, synthetic construct
GGSGVDFFL

SEQ ID NO: 20852 - protein, 9 aa, synthetic construct
GGAGIDVVE

SEQ ID NO: 20853 - protein, 9 aa, synthetic construct
GGAGIDWFI

SEQ ID NO: 20854 - protein, 9 aa, synthetic construct
GGSGVDDMI

SEQ ID NO: 20855 - protein, 9 aa, synthetic construct
GGFGDDYMS

SEQ ID NO: 20856 - protein, 9 aa, synthetic construct
GGSGVDDLD

SEQ ID NO: 20857 - protein, 9 aa, synthetic construct
GGFGEDDIQ

SEQ ID NO: 20858 - protein, 9 aa, synthetic construct
GGSGVDAMS

SEQ ID NO: 20859 - protein, 9 aa, synthetic construct
GGSGVDAMN

SEQ ID NO: 20860 - protein, 9 aa, synthetic construct
GGEGNDELG

SEQ ID NO: 20861 - protein, 9 aa, synthetic construct
GGSGVDALV

SEQ ID NO: 20862 - protein, 9 aa, synthetic construct
GGAGIDWYY

SEQ ID NO: 20863 - protein, 9 aa, synthetic construct
GGSGTDYLS

SEQ ID NO: 20864 - protein, 9 aa, synthetic construct
GGAGIDYLD

SEQ ID NO: 20865 - protein, 9 aa, synthetic construct
GGFGEDLFK

SEQ ID NO: 20866 - protein, 9 aa, synthetic construct
GGAGIDYLV

SEQ ID NO: 20867 - protein, 9 aa, synthetic construct
GGSGTDVLR

SEQ ID NO: 20868 - protein, 9 aa, synthetic construct
GGEGNDEII

SEQ ID NO: 20869 - protein, 9 aa, synthetic construct
GGSGTDVLE

SEQ ID NO: 20870 - protein, 9 aa, synthetic construct
GGSGTDVAQ

SEQ ID NO: 20871 - protein, 9 aa, synthetic construct
GGFGEDQLY

SEQ ID NO: 20872 - protein, 9 aa, synthetic construct
GGSGTDTVW

SEQ ID NO: 20873 - protein, 9 aa, synthetic construct
GGFGDDYII

SEQ ID NO: 20874 - protein, 9 aa, synthetic construct
GGEGNDELL

SEQ ID NO: 20875 - protein, 9 aa, synthetic construct
GGTGADHME

SEQ ID NO: 20876 - protein, 9 aa, synthetic construct
GGFGDDWLG

SEQ ID NO: 20877 - protein, 9 aa, synthetic construct
GGAGIDTIY

SEQ ID NO: 20878 - protein, 9 aa, synthetic construct
GGSGVDSLY

SEQ ID NO: 20879 - protein, 9 aa, synthetic construct
GGSGVDSAI

SEQ ID NO: 20880 - protein, 9 aa, synthetic construct
GGFGDDVLL

SEQ ID NO: 20881 - protein, 9 aa, synthetic construct
GGAGIDTLQ

SEQ ID NO: 20882 - protein, 9 aa, synthetic construct
GGSGVDRLF

SEQ ID NO: 20883 - protein, 9 aa, synthetic construct
GGSGVDRLA

SEQ ID NO: 20884 - protein, 9 aa, synthetic construct
GGSGVDRID

SEQ ID NO: 20885 - protein, 9 aa, synthetic construct
GGSGVDQMF

SEQ ID NO: 20886 - protein, 9 aa, synthetic construct
GGSGVDQLE

SEQ ID NO: 20887 - protein, 9 aa, synthetic construct
GGSGVDQIW

SEQ ID NO: 20888 - protein, 9 aa, synthetic construct
GGSGVDQID

SEQ ID NO: 20889 - protein, 9 aa, synthetic construct
GGFGDDVLR

SEQ ID NO: 20890 - protein, 9 aa, synthetic construct
GGAGIDTVG

SEQ ID NO: 20891 - protein, 9 aa, synthetic construct
GGFGDDVLY

SEQ ID NO: 20892 - protein, 9 aa, synthetic construct
GGSGVDLMI

SEQ ID NO: 20893 - protein, 9 aa, synthetic construct
GGFGDDVMT

SEQ ID NO: 20894 - protein, 9 aa, synthetic construct
GGSGVDLLE

SEQ ID NO: 20895 - protein, 9 aa, synthetic construct
GGSGVDLIY

SEQ ID NO: 20896 - protein, 9 aa, synthetic construct
GGAGIDVID

SEQ ID NO: 20897 - protein, 9 aa, synthetic construct
GGAGIDVIT

SEQ ID NO: 20898 - protein, 9 aa, synthetic construct
GGSGVDIMT

SEQ ID NO: 20899 - protein, 9 aa, synthetic construct
GGSGVDILD

SEQ ID NO: 20900 - protein, 9 aa, synthetic construct
GGSGVDIIS

SEQ ID NO: 20901 - protein, 9 aa, synthetic construct
GGSGVDIAD

SEQ ID NO: 20902 - protein, 9 aa, synthetic construct
GGSGTDTVD

SEQ ID NO: 20903 - protein, 9 aa, synthetic construct
GGFGEDRLA

SEQ ID NO: 20904 - protein, 9 aa, synthetic construct
GGEGNDEID

SEQ ID NO: 20905 - protein, 9 aa, synthetic construct
GGFGEDSIR

SEQ ID NO: 20906 - protein, 9 aa, synthetic construct
GGFGFDQLN

SEQ ID NO: 20907 - protein, 9 aa, synthetic construct
GGFGFDQLV

SEQ ID NO: 20908 - protein, 9 aa, synthetic construct
GGFGFDRLA

SEQ ID NO: 20909 - protein, 9 aa, synthetic construct
GGSGTDILE

SEQ ID NO: 20910 - protein, 9 aa, synthetic construct
GGEGNDDIV

SEQ ID NO: 20911 - protein, 9 aa, synthetic construct
GGSGTDIAD

SEQ ID NO: 20912 - protein, 9 aa, synthetic construct
GGAGKDHLD

SEQ ID NO: 20913 - protein, 9 aa, synthetic construct
GGEGNDDIL

SEQ ID NO: 20914 - protein, 9 aa, synthetic construct
GGAGKDHLL

SEQ ID NO: 20915 - protein, 9 aa, synthetic construct
GGAGKDIFK

SEQ ID NO: 20916 - protein, 9 aa, synthetic construct
GGAGKDIIA

SEQ ID NO: 20917 - protein, 9 aa, synthetic construct
GGAGKDIID

SEQ ID NO: 20918 - protein, 9 aa, synthetic construct
GGAGKDIIY

SEQ ID NO: 20919 - protein, 9 aa, synthetic construct
GGAGKDILD

SEQ ID NO: 20920 - protein, 9 aa, synthetic construct
GGSGTDDLR

SEQ ID NO: 20921 - protein, 9 aa, synthetic construct
GGAGKDILL

SEQ ID NO: 20922 - protein, 9 aa, synthetic construct
GGSGTDALN

SEQ ID NO: 20923 - protein, 9 aa, synthetic construct
GGAGKDILR

SEQ ID NO: 20924 - protein, 9 aa, synthetic construct
GGSGSDYLF

SEQ ID NO: 20925 - protein, 9 aa, synthetic construct
GGSGSDYLC

SEQ ID NO: 20926 - protein, 9 aa, synthetic construct
GGSGSDYIN

SEQ ID NO: 20927 - protein, 9 aa, synthetic construct
GGSGSDYIL

SEQ ID NO: 20928 - protein, 9 aa, synthetic construct
GGSGSDYIE

SEQ ID NO: 20929 - protein, 9 aa, synthetic construct
GGAGKDIML

SEQ ID NO: 20930 - protein, 9 aa, synthetic construct
GGSGSDWLF

SEQ ID NO: 20931 - protein, 9 aa, synthetic construct
GGSGTDKLY

SEQ ID NO: 20932 - protein, 9 aa, synthetic construct
GGSGTDLIE

SEQ ID NO: 20933 - protein, 9 aa, synthetic construct
GGEGNDDLD

SEQ ID NO: 20934 - protein, 9 aa, synthetic construct
GGEGNDDLR

SEQ ID NO: 20935 - protein, 9 aa, synthetic construct
GGEGNDEFV

SEQ ID NO: 20936 - protein, 9 aa, synthetic construct
GGSGTDTIV

SEQ ID NO: 20937 - protein, 9 aa, synthetic construct
GGSGTDTIT

SEQ ID NO: 20938 - protein, 9 aa, synthetic construct
GGSGTDTIN

SEQ ID NO: 20939 - protein, 9 aa, synthetic construct
GGSGTDTII

SEQ ID NO: 20940 - protein, 9 aa, synthetic construct
GGSGTDTFD

SEQ ID NO: 20941 - protein, 9 aa, synthetic construct
GGFGEDTLE

SEQ ID NO: 20942 - protein, 9 aa, synthetic construct
GGSGTDSMI

SEQ ID NO: 20943 - protein, 9 aa, synthetic construct
GGEGNDDLT

SEQ ID NO: 20944 - protein, 9 aa, synthetic construct
GGSGTDSLI

SEQ ID NO: 20945 - protein, 9 aa, synthetic construct
GGSGTDSLD

SEQ ID NO: 20946 - protein, 9 aa, synthetic construct
GGSGTDSID

SEQ ID NO: 20947 - protein, 9 aa, synthetic construct
GGSGTDLLS

SEQ ID NO: 20948 - protein, 9 aa, synthetic construct
GGSGTDRLN

SEQ ID NO: 20949 - protein, 9 aa, synthetic construct
GGEGNDDLK

SEQ ID NO: 20950 - protein, 9 aa, synthetic construct
GGAGKDELF

SEQ ID NO: 20951 - protein, 9 aa, synthetic construct
GGSGTDQLY

SEQ ID NO: 20952 - protein, 9 aa, synthetic construct
GGAGKDELI

SEQ ID NO: 20953 - protein, 9 aa, synthetic construct
GGSGTDQIL

SEQ ID NO: 20954 - protein, 9 aa, synthetic construct
GGFGEDVIR

SEQ ID NO: 20955 - protein, 9 aa, synthetic construct
GGSGTDNFY

SEQ ID NO: 20956 - protein, 9 aa, synthetic construct
GGFGEDYVD

SEQ ID NO: 20957 - protein, 9 aa, synthetic construct
GGSGTDMLD

SEQ ID NO: 20958 - protein, 9 aa, synthetic construct
GGFGFDFLY

SEQ ID NO: 20959 - protein, 9 aa, synthetic construct
GGSGVDTAG

SEQ ID NO: 20960 - protein, 9 aa, synthetic construct
GGSGVDTAR

SEQ ID NO: 20961 - protein, 9 aa, synthetic construct
GGSGVDTAV

SEQ ID NO: 20962 - protein, 9 aa, synthetic construct
GGFGDDTMS

SEQ ID NO: 20963 - protein, 9 aa, synthetic construct
GGFGDDTIT

SEQ ID NO: 20964 - protein, 9 aa, synthetic construct
GGTGADDIS

SEQ ID NO: 20965 - protein, 9 aa, synthetic construct
GGFGDDTLE

SEQ ID NO: 20966 - protein, 9 aa, synthetic construct
GGTGADDID

SEQ ID NO: 20967 - protein, 9 aa, synthetic construct
GGAGIDQLT

SEQ ID NO: 20968 - protein, 9 aa, synthetic construct
GGTGADAME

SEQ ID NO: 20969 - protein, 9 aa, synthetic construct
GGAGIDRAD

SEQ ID NO: 20970 - protein, 9 aa, synthetic construct
GGAGIDRAL

SEQ ID NO: 20971 - protein, 9 aa, synthetic construct
GGTGADALH

SEQ ID NO: 20972 - protein, 9 aa, synthetic construct
GGTGADAIY

SEQ ID NO: 20973 - protein, 9 aa, synthetic construct
GGFGDDTLR

SEQ ID NO: 20974 - protein, 9 aa, synthetic construct
GGFGDDTLS

SEQ ID NO: 20975 - protein, 9 aa, synthetic construct
GGTGADAIF

SEQ ID NO: 20976 - protein, 9 aa, synthetic construct
GGTGADAIA

SEQ ID NO: 20977 - protein, 9 aa, synthetic construct
GGTGADAFV

SEQ ID NO: 20978 - protein, 9 aa, synthetic construct
GGAGIDRIT

SEQ ID NO: 20979 - protein, 9 aa, synthetic construct
GGSGYDYFY

SEQ ID NO: 20980 - protein, 9 aa, synthetic construct
GGAGIDRLD

SEQ ID NO: 20981 - protein, 9 aa, synthetic construct
GGSGYDVLN

SEQ ID NO: 20982 - protein, 9 aa, synthetic construct
GGSGYDTVE

SEQ ID NO: 20983 - protein, 9 aa, synthetic construct
GGSGYDTMI

SEQ ID NO: 20984 - protein, 9 aa, synthetic construct
GGSGYDTLI

SEQ ID NO: 20985 - protein, 9 aa, synthetic construct
GGSGYDTLD

SEQ ID NO: 20986 - protein, 9 aa, synthetic construct
GGSGYDTIY

SEQ ID NO: 20987 - protein, 9 aa, synthetic construct
GGFGDDTMR

SEQ ID NO: 20988 - protein, 9 aa, synthetic construct
GGEGNDFIY

SEQ ID NO: 20989 - protein, 9 aa, synthetic construct
GGTGADDLQ

SEQ ID NO: 20990 - protein, 9 aa, synthetic construct
GGTGADDLY

SEQ ID NO: 20991 - protein, 9 aa, synthetic construct
GGTGADEMV

SEQ ID NO: 20992 - protein, 9 aa, synthetic construct
GGTGADHLR

SEQ ID NO: 20993 - protein, 9 aa, synthetic construct
GGAGIDLLR

SEQ ID NO: 20994 - protein, 9 aa, synthetic construct
GGAGIDLLT

SEQ ID NO: 20995 - protein, 9 aa, synthetic construct
GGTGADGLL

SEQ ID NO: 20996 - protein, 9 aa, synthetic construct
GGFGDDSLT

SEQ ID NO: 20997 - protein, 9 aa, synthetic construct
GGEGNDFLN

SEQ ID NO: 20998 - protein, 9 aa, synthetic construct
GGFGDDSMN

SEQ ID NO: 20999 - protein, 9 aa, synthetic construct
GGEGNDFLL

SEQ ID NO: 21000 - protein, 9 aa, synthetic construct
GGTGADFLD

SEQ ID NO: 21001 - protein, 9 aa, synthetic construct
GGTGADFLA

SEQ ID NO: 21002 - protein, 9 aa, synthetic construct
GGFGDDTFL

SEQ ID NO: 21003 - protein, 9 aa, synthetic construct
GGTGADEMQ

SEQ ID NO: 21004 - protein, 9 aa, synthetic construct
GGTGADDMD

SEQ ID NO: 21005 - protein, 9 aa, synthetic construct
GGTGADEML

SEQ ID NO: 21006 - protein, 9 aa, synthetic construct
GGTGADEMI

SEQ ID NO: 21007 - protein, 9 aa, synthetic construct
GGTGADELV

SEQ ID NO: 21008 - protein, 9 aa, synthetic construct
GGTGADELS

SEQ ID NO: 21009 - protein, 9 aa, synthetic construct
GGAGIDNFV

SEQ ID NO: 21010 - protein, 9 aa, synthetic construct
GGTGADELF

SEQ ID NO: 21011 - protein, 9 aa, synthetic construct
GGTGADELD

SEQ ID NO: 21012 - protein, 9 aa, synthetic construct
GGTGADEIW

SEQ ID NO: 21013 - protein, 9 aa, synthetic construct
GGAGIDNLD

SEQ ID NO: 21014 - protein, 9 aa, synthetic construct
GGTGADEIA

SEQ ID NO: 21015 - protein, 9 aa, synthetic construct
GGFGDDTIH

SEQ ID NO: 21016 - protein, 9 aa, synthetic construct
GGAGIDRME

SEQ ID NO: 21017 - protein, 9 aa, synthetic construct
GGAGIDRMI

SEQ ID NO: 21018 - protein, 9 aa, synthetic construct
GGAGIDTIV

SEQ ID NO: 21019 - protein, 9 aa, synthetic construct
GGAGIDRML

SEQ ID NO: 21020 - protein, 9 aa, synthetic construct
GGSGWDRIE

SEQ ID NO: 21021 - protein, 9 aa, synthetic construct
GGAGIDSVY

SEQ ID NO: 21022 - protein, 9 aa, synthetic construct
GGSGWDMVS

SEQ ID NO: 21023 - protein, 9 aa, synthetic construct
GGFGDDVIA

SEQ ID NO: 21024 - protein, 9 aa, synthetic construct
GGSGWDLID

SEQ ID NO: 21025 - protein, 9 aa, synthetic construct
GGFGDDVID

SEQ ID NO: 21026 - protein, 9 aa, synthetic construct
GGAGIDTAE

SEQ ID NO: 21027 - protein, 9 aa, synthetic construct
GGSGVDYLY

SEQ ID NO: 21028 - protein, 9 aa, synthetic construct
GGSGVDYLS

SEQ ID NO: 21029 - protein, 9 aa, synthetic construct
GGSGVDYLC

SEQ ID NO: 21030 - protein, 9 aa, synthetic construct
GGSGVDYFN

SEQ ID NO: 21031 - protein, 9 aa, synthetic construct
GGSGVDWLD

SEQ ID NO: 21032 - protein, 9 aa, synthetic construct
GGAGIDTAN

SEQ ID NO: 21033 - protein, 9 aa, synthetic construct
GGSGVDVLL

SEQ ID NO: 21034 - protein, 9 aa, synthetic construct
GGSGVDVFR

SEQ ID NO: 21035 - protein, 9 aa, synthetic construct
GGSGVDTVT

SEQ ID NO: 21036 - protein, 9 aa, synthetic construct
GGSGVDTVS

SEQ ID NO: 21037 - protein, 9 aa, synthetic construct
GGSGVDTVI

SEQ ID NO: 21038 - protein, 9 aa, synthetic construct
GGAGIDTFL

SEQ ID NO: 21039 - protein, 9 aa, synthetic construct
GGFGDDVLH

SEQ ID NO: 21040 - protein, 9 aa, synthetic construct
GGAGIDTIH

SEQ ID NO: 21041 - protein, 9 aa, synthetic construct
GGSGVDTIT

SEQ ID NO: 21042 - protein, 9 aa, synthetic construct
GGSGVDTIK

SEQ ID NO: 21043 - protein, 9 aa, synthetic construct
GGAGIDTIQ

SEQ ID NO: 21044 - protein, 9 aa, synthetic construct
GGSGVDTFF

SEQ ID NO: 21045 - protein, 9 aa, synthetic construct
GGSGWDRVN

SEQ ID NO: 21046 - protein, 9 aa, synthetic construct
GGSGWDSAH

SEQ ID NO: 21047 - protein, 9 aa, synthetic construct
GGEGNDEVY

SEQ ID NO: 21048 - protein, 9 aa, synthetic construct
GGFGDDTVS

SEQ ID NO: 21049 - protein, 9 aa, synthetic construct
GGAGIDRMS

SEQ ID NO: 21050 - protein, 9 aa, synthetic construct
GGSGYDRLT

SEQ ID NO: 21051 - protein, 9 aa, synthetic construct
GGSGYDRFL

SEQ ID NO: 21052 - protein, 9 aa, synthetic construct
GGAGIDRVT

SEQ ID NO: 21053 - protein, 9 aa, synthetic construct
GGAGIDSAD

SEQ ID NO: 21054 - protein, 9 aa, synthetic construct
GGFGDDTVL

SEQ ID NO: 21055 - protein, 9 aa, synthetic construct
GGSGYDMLY

SEQ ID NO: 21056 - protein, 9 aa, synthetic construct
GGAGIDSAT

SEQ ID NO: 21057 - protein, 9 aa, synthetic construct
GGAGIDSFV

SEQ ID NO: 21058 - protein, 9 aa, synthetic construct
GGSGYDIYQ

SEQ ID NO: 21059 - protein, 9 aa, synthetic construct
GGAGIDSIG

SEQ ID NO: 21060 - protein, 9 aa, synthetic construct
GGEGNDFII

SEQ ID NO: 21061 - protein, 9 aa, synthetic construct
GGAGIDSMS

SEQ ID NO: 21062 - protein, 9 aa, synthetic construct
GGSGYDGLY

SEQ ID NO: 21063 - protein, 9 aa, synthetic construct
GGSGYDGLN

SEQ ID NO: 21064 - protein, 9 aa, synthetic construct
GGAGIDSLL

SEQ ID NO: 21065 - protein, 9 aa, synthetic construct
GGSGYDEIY

SEQ ID NO: 21066 - protein, 9 aa, synthetic construct
GGEGNDFAF

SEQ ID NO: 21067 - protein, 9 aa, synthetic construct
GGAGIDSLW

SEQ ID NO: 21068 - protein, 9 aa, synthetic construct
GGSGWDVLT

SEQ ID NO: 21069 - protein, 9 aa, synthetic construct
GGAGIDSMA

SEQ ID NO: 21070 - protein, 9 aa, synthetic construct
GGFGDDVFL

SEQ ID NO: 21071 - protein, 9 aa, synthetic construct
GGSGWDTLE

SEQ ID NO: 21072 - protein, 9 aa, synthetic construct
GGSGWDTLD

SEQ ID NO: 21073 - protein, 9 aa, synthetic construct
GGSGSDWLD

SEQ ID NO: 21074 - protein, 9 aa, synthetic construct
GGFGFDSID

SEQ ID NO: 21075 - protein, 9 aa, synthetic construct
GGSGSDWAS

SEQ ID NO: 21076 - protein, 9 aa, synthetic construct
GGSGRDSLR

SEQ ID NO: 21077 - protein, 9 aa, synthetic construct
GGAGKDTAL

SEQ ID NO: 21078 - protein, 9 aa, synthetic construct
GGSGSDAIS

SEQ ID NO: 21079 - protein, 9 aa, synthetic construct
GGEGMDVFV

SEQ ID NO: 21080 - protein, 9 aa, synthetic construct
GGAGKDTAS

SEQ ID NO: 21081 - protein, 9 aa, synthetic construct
GGAGKDTAV

SEQ ID NO: 21082 - protein, 9 aa, synthetic construct
GGSGRDYME

SEQ ID NO: 21083 - protein, 9 aa, synthetic construct
GGSGRDYLK

SEQ ID NO: 21084 - protein, 9 aa, synthetic construct
GGSGRDYAV

SEQ ID NO: 21085 - protein, 9 aa, synthetic construct
GGEGMDTVD

SEQ ID NO: 21086 - protein, 9 aa, synthetic construct
GGSGRDWID

SEQ ID NO: 21087 - protein, 9 aa, synthetic construct
GGSGRDWAD

SEQ ID NO: 21088 - protein, 9 aa, synthetic construct
GGAGKDTIN

SEQ ID NO: 21089 - protein, 9 aa, synthetic construct
GGAGKDTIR

SEQ ID NO: 21090 - protein, 9 aa, synthetic construct
GGSGRDVLA

SEQ ID NO: 21091 - protein, 9 aa, synthetic construct
GGSGRDVIS

SEQ ID NO: 21092 - protein, 9 aa, synthetic construct
GGSGRDVID

SEQ ID NO: 21093 - protein, 9 aa, synthetic construct
GGSGRDVFT

SEQ ID NO: 21094 - protein, 9 aa, synthetic construct
GGSGRDTYS

SEQ ID NO: 21095 - protein, 9 aa, synthetic construct
GGSGRDTMV

SEQ ID NO: 21096 - protein, 9 aa, synthetic construct
GGSGRDTLV

SEQ ID NO: 21097 - protein, 9 aa, synthetic construct
GGSGRDTLH

SEQ ID NO: 21098 - protein, 9 aa, synthetic construct
GGEGMDSLI

SEQ ID NO: 21099 - protein, 9 aa, synthetic construct
GGSGRDTIG

SEQ ID NO: 21100 - protein, 9 aa, synthetic construct
GGSGRDTIE

SEQ ID NO: 21101 - protein, 9 aa, synthetic construct
GGAGKDTLW

SEQ ID NO: 21102 - protein, 9 aa, synthetic construct
GGSGSDALD

SEQ ID NO: 21103 - protein, 9 aa, synthetic construct
GGSGSDALE

SEQ ID NO: 21104 - protein, 9 aa, synthetic construct
GGFGHDTVF

SEQ ID NO: 21105 - protein, 9 aa, synthetic construct
GGSGSDELE

SEQ ID NO: 21106 - protein, 9 aa, synthetic construct
GGAGKDRVF

SEQ ID NO: 21107 - protein, 9 aa, synthetic construct
GGEGNDAIF

SEQ ID NO: 21108 - protein, 9 aa, synthetic construct
GGAGKDSFI

SEQ ID NO: 21109 - protein, 9 aa, synthetic construct
GGSGSDFLD

SEQ ID NO: 21110 - protein, 9 aa, synthetic construct
GGAGKDSFR

SEQ ID NO: 21111 - protein, 9 aa, synthetic construct
GGAGKDSIF

SEQ ID NO: 21112 - protein, 9 aa, synthetic construct
GGAGKDSIG

SEQ ID NO: 21113 - protein, 9 aa, synthetic construct
GGSGSDELR

SEQ ID NO: 21114 - protein, 9 aa, synthetic construct
GGSGSDELI

SEQ ID NO: 21115 - protein, 9 aa, synthetic construct
GGSGSDELH

SEQ ID NO: 21116 - protein, 9 aa, synthetic construct
GGSGSDELF

SEQ ID NO: 21117 - protein, 9 aa, synthetic construct
GGSGSDELD

SEQ ID NO: 21118 - protein, 9 aa, synthetic construct
GGFGHDTLS

SEQ ID NO: 21119 - protein, 9 aa, synthetic construct
GGAGKDSLN

SEQ ID NO: 21120 - protein, 9 aa, synthetic construct
GGEGNDAID

SEQ ID NO: 21121 - protein, 9 aa, synthetic construct
GGSGSDDLR

SEQ ID NO: 21122 - protein, 9 aa, synthetic construct
GGSGSDDLN

SEQ ID NO: 21123 - protein, 9 aa, synthetic construct
GGAGKDSLV

SEQ ID NO: 21124 - protein, 9 aa, synthetic construct
GGAGKDSMA

SEQ ID NO: 21125 - protein, 9 aa, synthetic construct
GGSGSDDIA

SEQ ID NO: 21126 - protein, 9 aa, synthetic construct
GGAGKDSMD

SEQ ID NO: 21127 - protein, 9 aa, synthetic construct
GGSGSDAVF

SEQ ID NO: 21128 - protein, 9 aa, synthetic construct
GGAGKDSMT

SEQ ID NO: 21129 - protein, 9 aa, synthetic construct
GGEGMDVLY

SEQ ID NO: 21130 - protein, 9 aa, synthetic construct
GGFGIDQLS

SEQ ID NO: 21131 - protein, 9 aa, synthetic construct
GGSGRDSLK

SEQ ID NO: 21132 - protein, 9 aa, synthetic construct
GGSGSDFYV

SEQ ID NO: 21133 - protein, 9 aa, synthetic construct
GGSGRDSLF

SEQ ID NO: 21134 - protein, 9 aa, synthetic construct
GGSGRDKLS

SEQ ID NO: 21135 - protein, 9 aa, synthetic construct
GGSGRDKLR

SEQ ID NO: 21136 - protein, 9 aa, synthetic construct
GGSGRDKLD

SEQ ID NO: 21137 - protein, 9 aa, synthetic construct
GGEGLDYLT

SEQ ID NO: 21138 - protein, 9 aa, synthetic construct
GGSGRDIVI

SEQ ID NO: 21139 - protein, 9 aa, synthetic construct
GGFGKDTVS

SEQ ID NO: 21140 - protein, 9 aa, synthetic construct
GGFGKDVIT

SEQ ID NO: 21141 - protein, 9 aa, synthetic construct
GGFGKDVLS

SEQ ID NO: 21142 - protein, 9 aa, synthetic construct
GGSGRDILR

SEQ ID NO: 21143 - protein, 9 aa, synthetic construct
GGEGLDYAI

SEQ ID NO: 21144 - protein, 9 aa, synthetic construct
GGSGRDILL

SEQ ID NO: 21145 - protein, 9 aa, synthetic construct
GGAGKDWLY

SEQ ID NO: 21146 - protein, 9 aa, synthetic construct
GGFGLDLLY

SEQ ID NO: 21147 - protein, 9 aa, synthetic construct
GGSGRDGLF

SEQ ID NO: 21148 - protein, 9 aa, synthetic construct
GGSGRDGFV

SEQ ID NO: 21149 - protein, 9 aa, synthetic construct
GGAGKDYFI

SEQ ID NO: 21150 - protein, 9 aa, synthetic construct
GGAGKDYIT

SEQ ID NO: 21151 - protein, 9 aa, synthetic construct
GGSGRDFLN

SEQ ID NO: 21152 - protein, 9 aa, synthetic construct
GGAGKDYLW

SEQ ID NO: 21153 - protein, 9 aa, synthetic construct
GGAGKDYLY

SEQ ID NO: 21154 - protein, 9 aa, synthetic construct
GGFGLDTAL

SEQ ID NO: 21155 - protein, 9 aa, synthetic construct
GGSGRDELI

SEQ ID NO: 21156 - protein, 9 aa, synthetic construct
GGSGRDELF

SEQ ID NO: 21157 - protein, 9 aa, synthetic construct
GGAGLDAFR

SEQ ID NO: 21158 - protein, 9 aa, synthetic construct
GGSGRDEIF

SEQ ID NO: 21159 - protein, 9 aa, synthetic construct
GGSGRDKLV

SEQ ID NO: 21160 - protein, 9 aa, synthetic construct
GGSGRDLAD

SEQ ID NO: 21161 - protein, 9 aa, synthetic construct
GGSGRDLLA

SEQ ID NO: 21162 - protein, 9 aa, synthetic construct
GGSGRDQLY

SEQ ID NO: 21163 - protein, 9 aa, synthetic construct
GGEGMDLLT

SEQ ID NO: 21164 - protein, 9 aa, synthetic construct
GGSGRDSIL

SEQ ID NO: 21165 - protein, 9 aa, synthetic construct
GGAGKDTYT

SEQ ID NO: 21166 - protein, 9 aa, synthetic construct
GGSGRDRMY

SEQ ID NO: 21167 - protein, 9 aa, synthetic construct
GGAGKDVFI

SEQ ID NO: 21168 - protein, 9 aa, synthetic construct
GGSGRDRLN

SEQ ID NO: 21169 - protein, 9 aa, synthetic construct
GGSGRDRIY

SEQ ID NO: 21170 - protein, 9 aa, synthetic construct
GGSGRDRIS

SEQ ID NO: 21171 - protein, 9 aa, synthetic construct
GGSGRDRIF

SEQ ID NO: 21172 - protein, 9 aa, synthetic construct
GGSGRDRFV

SEQ ID NO: 21173 - protein, 9 aa, synthetic construct
GGAGKDVFN

SEQ ID NO: 21174 - protein, 9 aa, synthetic construct
GGEGMDIFK

SEQ ID NO: 21175 - protein, 9 aa, synthetic construct
GGSGRDLLE

SEQ ID NO: 21176 - protein, 9 aa, synthetic construct
GGFGKDILF

SEQ ID NO: 21177 - protein, 9 aa, synthetic construct
GGAGKDVIL

SEQ ID NO: 21178 - protein, 9 aa, synthetic construct
GGSGRDQIR

SEQ ID NO: 21179 - protein, 9 aa, synthetic construct
GGSGRDQFK

SEQ ID NO: 21180 - protein, 9 aa, synthetic construct
GGAGKDVIQ

SEQ ID NO: 21181 - protein, 9 aa, synthetic construct
GGSGRDNLI

SEQ ID NO: 21182 - protein, 9 aa, synthetic construct
GGSGRDMLS

SEQ ID NO: 21183 - protein, 9 aa, synthetic construct
GGAGKDVIY

SEQ ID NO: 21184 - protein, 9 aa, synthetic construct
GGAGKDVLA

SEQ ID NO: 21185 - protein, 9 aa, synthetic construct
GGSGRDLLY

SEQ ID NO: 21186 - protein, 9 aa, synthetic construct
GGFGKDTLI

SEQ ID NO: 21187 - protein, 9 aa, synthetic construct
GGSGSDFYL

SEQ ID NO: 21188 - protein, 9 aa, synthetic construct
GGFGHDRLH

SEQ ID NO: 21189 - protein, 9 aa, synthetic construct
GGSGSDVYN

SEQ ID NO: 21190 - protein, 9 aa, synthetic construct
GGSGSDQLY

SEQ ID NO: 21191 - protein, 9 aa, synthetic construct
GGSGSDSLQ

SEQ ID NO: 21192 - protein, 9 aa, synthetic construct
GGSGSDSLN

SEQ ID NO: 21193 - protein, 9 aa, synthetic construct
GGSGSDSLM

SEQ ID NO: 21194 - protein, 9 aa, synthetic construct
GGSGSDSLI

SEQ ID NO: 21195 - protein, 9 aa, synthetic construct
GGSGSDSLE

SEQ ID NO: 21196 - protein, 9 aa, synthetic construct
GGAGKDLFQ

SEQ ID NO: 21197 - protein, 9 aa, synthetic construct
GGSGSDSIS

SEQ ID NO: 21198 - protein, 9 aa, synthetic construct
GGAGKDLFY

SEQ ID NO: 21199 - protein, 9 aa, synthetic construct
GGSGSDSIE

SEQ ID NO: 21200 - protein, 9 aa, synthetic construct
GGSGSDSFV

SEQ ID NO: 21201 - protein, 9 aa, synthetic construct
GGAGKDLID

SEQ ID NO: 21202 - protein, 9 aa, synthetic construct
GGAGKDLIE

SEQ ID NO: 21203 - protein, 9 aa, synthetic construct
GGSGSDRMN

SEQ ID NO: 21204 - protein, 9 aa, synthetic construct
GGSGSDRML

SEQ ID NO: 21205 - protein, 9 aa, synthetic construct
GGSGSDRMI

SEQ ID NO: 21206 - protein, 9 aa, synthetic construct
GGAGKDLIN

SEQ ID NO: 21207 - protein, 9 aa, synthetic construct
GGSGSDRLI

SEQ ID NO: 21208 - protein, 9 aa, synthetic construct
GGFGGDDLF

SEQ ID NO: 21209 - protein, 9 aa, synthetic construct
GGEGNDALQ

SEQ ID NO: 21210 - protein, 9 aa, synthetic construct
GGSGSDRIF

SEQ ID NO: 21211 - protein, 9 aa, synthetic construct
GGAGKDLLK

SEQ ID NO: 21212 - protein, 9 aa, synthetic construct
GGAGKDLLR

SEQ ID NO: 21213 - protein, 9 aa, synthetic construct
GGSGSDQVF

SEQ ID NO: 21214 - protein, 9 aa, synthetic construct
GGSGSDQMV

SEQ ID NO: 21215 - protein, 9 aa, synthetic construct
GGFGGDRLF

SEQ ID NO: 21216 - protein, 9 aa, synthetic construct
GGSGSDSMV

SEQ ID NO: 21217 - protein, 9 aa, synthetic construct
GGEGNDALV

SEQ ID NO: 21218 - protein, 9 aa, synthetic construct
GGAGKDKVT

SEQ ID NO: 21219 - protein, 9 aa, synthetic construct
GGSGSDTYH

SEQ ID NO: 21220 - protein, 9 aa, synthetic construct
GGSGSDVYL

SEQ ID NO: 21221 - protein, 9 aa, synthetic construct
GGSGSDVVL

SEQ ID NO: 21222 - protein, 9 aa, synthetic construct
GGSGSDVLY

SEQ ID NO: 21223 - protein, 9 aa, synthetic construct
GGSGSDVLL

SEQ ID NO: 21224 - protein, 9 aa, synthetic construct
GGSGSDVIL

SEQ ID NO: 21225 - protein, 9 aa, synthetic construct
GGSGSDVII

SEQ ID NO: 21226 - protein, 9 aa, synthetic construct
GGSGSDVID

SEQ ID NO: 21227 - protein, 9 aa, synthetic construct
GGSGSDVFK

SEQ ID NO: 21228 - protein, 9 aa, synthetic construct
GGSGSDVAV

SEQ ID NO: 21229 - protein, 9 aa, synthetic construct
GGSGSDTYY

SEQ ID NO: 21230 - protein, 9 aa, synthetic construct
GGFGFDTIE

SEQ ID NO: 21231 - protein, 9 aa, synthetic construct
GGAGKDKIY

SEQ ID NO: 21232 - protein, 9 aa, synthetic construct
GGFGFDWAT

SEQ ID NO: 21233 - protein, 9 aa, synthetic construct
GGSGSDTVL

SEQ ID NO: 21234 - protein, 9 aa, synthetic construct
GGAGKDKLD

SEQ ID NO: 21235 - protein, 9 aa, synthetic construct
GGSGSDTMW

SEQ ID NO: 21236 - protein, 9 aa, synthetic construct
GGAGKDKLE

SEQ ID NO: 21237 - protein, 9 aa, synthetic construct
GGEGNDAVR

SEQ ID NO: 21238 - protein, 9 aa, synthetic construct
GGSGSDTLQ

SEQ ID NO: 21239 - protein, 9 aa, synthetic construct
GGSGSDTLM

SEQ ID NO: 21240 - protein, 9 aa, synthetic construct
GGAGKDKLL

SEQ ID NO: 21241 - protein, 9 aa, synthetic construct
GGSGSDTIS

SEQ ID NO: 21242 - protein, 9 aa, synthetic construct
GGSGSDTIH

SEQ ID NO: 21243 - protein, 9 aa, synthetic construct
GGSGSDTFL

SEQ ID NO: 21244 - protein, 9 aa, synthetic construct
GGAGKDLML

SEQ ID NO: 21245 - protein, 9 aa, synthetic construct
GGSGSDQLN

SEQ ID NO: 21246 - protein, 9 aa, synthetic construct
GGSGSDGLL

SEQ ID NO: 21247 - protein, 9 aa, synthetic construct
GGSGSDQLH

SEQ ID NO: 21248 - protein, 9 aa, synthetic construct
GGAGKDQMT

SEQ ID NO: 21249 - protein, 9 aa, synthetic construct
GGSGSDKIY

SEQ ID NO: 21250 - protein, 9 aa, synthetic construct
GGSGSDKIW

SEQ ID NO: 21251 - protein, 9 aa, synthetic construct
GGAGKDQVD

SEQ ID NO: 21252 - protein, 9 aa, synthetic construct
GGFGHDQLW

SEQ ID NO: 21253 - protein, 9 aa, synthetic construct
GGSGSDKFI

SEQ ID NO: 21254 - protein, 9 aa, synthetic construct
GGSGSDIYV

SEQ ID NO: 21255 - protein, 9 aa, synthetic construct
GGAGKDRIE

SEQ ID NO: 21256 - protein, 9 aa, synthetic construct
GGFGHDQLY

SEQ ID NO: 21257 - protein, 9 aa, synthetic construct
GGSGSDILY

SEQ ID NO: 21258 - protein, 9 aa, synthetic construct
GGAGKDRIN

SEQ ID NO: 21259 - protein, 9 aa, synthetic construct
GGSGSDILM

SEQ ID NO: 21260 - protein, 9 aa, synthetic construct
GGSGSDILL

SEQ ID NO: 21261 - protein, 9 aa, synthetic construct
GGEGNDAIS

SEQ ID NO: 21262 - protein, 9 aa, synthetic construct
GGAGKDRIY

SEQ ID NO: 21263 - protein, 9 aa, synthetic construct
GGSGSDIIN

SEQ ID NO: 21264 - protein, 9 aa, synthetic construct
GGAGKDRLH

SEQ ID NO: 21265 - protein, 9 aa, synthetic construct
GGSGSDIFA

SEQ ID NO: 21266 - protein, 9 aa, synthetic construct
GGSGSDIAD

SEQ ID NO: 21267 - protein, 9 aa, synthetic construct
GGAGKDRLK

SEQ ID NO: 21268 - protein, 9 aa, synthetic construct
GGSGSDHLR

SEQ ID NO: 21269 - protein, 9 aa, synthetic construct
GGAGKDRLS

SEQ ID NO: 21270 - protein, 9 aa, synthetic construct
GGSGSDHLF

SEQ ID NO: 21271 - protein, 9 aa, synthetic construct
GGAGKDRLY

SEQ ID NO: 21272 - protein, 9 aa, synthetic construct
GGSGSDGLR

SEQ ID NO: 21273 - protein, 9 aa, synthetic construct
GGFGHDQLE

SEQ ID NO: 21274 - protein, 9 aa, synthetic construct
GGSGSDKLI

SEQ ID NO: 21275 - protein, 9 aa, synthetic construct
GGSGSDKLK

SEQ ID NO: 21276 - protein, 9 aa, synthetic construct
GGAGKDNFF

SEQ ID NO: 21277 - protein, 9 aa, synthetic construct
GGSGSDQLF

SEQ ID NO: 21278 - protein, 9 aa, synthetic construct
GGSGSDQIF

SEQ ID NO: 21279 - protein, 9 aa, synthetic construct
GGAGKDMLD

SEQ ID NO: 21280 - protein, 9 aa, synthetic construct
GGSGSDNMA

SEQ ID NO: 21281 - protein, 9 aa, synthetic construct
GGAGKDMLI

SEQ ID NO: 21282 - protein, 9 aa, synthetic construct
GGSGSDNLV

SEQ ID NO: 21283 - protein, 9 aa, synthetic construct
GGSGSDNLS

SEQ ID NO: 21284 - protein, 9 aa, synthetic construct
GGAGKDMLL

SEQ ID NO: 21285 - protein, 9 aa, synthetic construct
GGSGSDNIY

SEQ ID NO: 21286 - protein, 9 aa, synthetic construct
GGSGSDNIN

SEQ ID NO: 21287 - protein, 9 aa, synthetic construct
GGSGSDNIA

SEQ ID NO: 21288 - protein, 9 aa, synthetic construct
GGEGNDALE

SEQ ID NO: 21289 - protein, 9 aa, synthetic construct
GGSGSDKLL

SEQ ID NO: 21290 - protein, 9 aa, synthetic construct
GGSGSDMLL

SEQ ID NO: 21291 - protein, 9 aa, synthetic construct
GGSGSDMLI

SEQ ID NO: 21292 - protein, 9 aa, synthetic construct
GGSGSDMID

SEQ ID NO: 21293 - protein, 9 aa, synthetic construct
GGFGHDEIH

SEQ ID NO: 21294 - protein, 9 aa, synthetic construct
GGFGHDFLD

SEQ ID NO: 21295 - protein, 9 aa, synthetic construct
GGAGKDQLD

SEQ ID NO: 21296 - protein, 9 aa, synthetic construct
GGFGHDIVN

SEQ ID NO: 21297 - protein, 9 aa, synthetic construct
GGSGSDLLK

SEQ ID NO: 21298 - protein, 9 aa, synthetic construct
GGSGSDLIT

SEQ ID NO: 21299 - protein, 9 aa, synthetic construct
GGSGSDLFV

SEQ ID NO: 21300 - protein, 9 aa, synthetic construct
GGSGSDLFE

SEQ ID NO: 21301 - protein, 9 aa, synthetic construct
GGAGIDLLL

SEQ ID NO: 21302 - protein, 9 aa, synthetic construct
GGTGADHMH

SEQ ID NO: 21303 - protein, 9 aa, synthetic construct
GGEGIDILV

SEQ ID NO: 21304 - protein, 9 aa, synthetic construct
GGTGDDWLI

SEQ ID NO: 21305 - protein, 9 aa, synthetic construct
GGTGDDWLG

SEQ ID NO: 21306 - protein, 9 aa, synthetic construct
GGTGDDWLE

SEQ ID NO: 21307 - protein, 9 aa, synthetic construct
GGTGDDWIY

SEQ ID NO: 21308 - protein, 9 aa, synthetic construct
GGTGDDVYF

SEQ ID NO: 21309 - protein, 9 aa, synthetic construct
GGAGHDILE

SEQ ID NO: 21310 - protein, 9 aa, synthetic construct
GGTGDDVVV

SEQ ID NO: 21311 - protein, 9 aa, synthetic construct
GGTGDDVVT

SEQ ID NO: 21312 - protein, 9 aa, synthetic construct
GGTGDDVMY

SEQ ID NO: 21313 - protein, 9 aa, synthetic construct
GGTGDDVMV

SEQ ID NO: 21314 - protein, 9 aa, synthetic construct
GGTGDDVMR

SEQ ID NO: 21315 - protein, 9 aa, synthetic construct
GGAGHDILN

SEQ ID NO: 21316 - protein, 9 aa, synthetic construct
GGAGHDILQ

SEQ ID NO: 21317 - protein, 9 aa, synthetic construct
GGAGHDILR

SEQ ID NO: 21318 - protein, 9 aa, synthetic construct
GGAGHDILV

SEQ ID NO: 21319 - protein, 9 aa, synthetic construct
GGTGDDVMA

SEQ ID NO: 21320 - protein, 9 aa, synthetic construct
GGTGDDVII

SEQ ID NO: 21321 - protein, 9 aa, synthetic construct
GGTGDDVIG

SEQ ID NO: 21322 - protein, 9 aa, synthetic construct
GGTGDDVIF

SEQ ID NO: 21323 - protein, 9 aa, synthetic construct
GGAGHDIVQ

SEQ ID NO: 21324 - protein, 9 aa, synthetic construct
GGTGDDVFA

SEQ ID NO: 21325 - protein, 9 aa, synthetic construct
GGTGDDTYS

SEQ ID NO: 21326 - protein, 9 aa, synthetic construct
GGFGADVAF

SEQ ID NO: 21327 - protein, 9 aa, synthetic construct
GGTGDDTYE

SEQ ID NO: 21328 - protein, 9 aa, synthetic construct
GGTGDDTYA

SEQ ID NO: 21329 - protein, 9 aa, synthetic construct
GGTGDDTVY

SEQ ID NO: 21330 - protein, 9 aa, synthetic construct
GGTGDDWLH

SEQ ID NO: 21331 - protein, 9 aa, synthetic construct
GGTGDDWLN

SEQ ID NO: 21332 - protein, 9 aa, synthetic construct
GGTGADHMI

SEQ ID NO: 21333 - protein, 9 aa, synthetic construct
GGAGHDILA

SEQ ID NO: 21334 - protein, 9 aa, synthetic construct
GGAGHDEIH

SEQ ID NO: 21335 - protein, 9 aa, synthetic construct
GGTGEDILI

SEQ ID NO: 21336 - protein, 9 aa, synthetic construct
GGFGADTIL

SEQ ID NO: 21337 - protein, 9 aa, synthetic construct
GGFGADTIQ

SEQ ID NO: 21338 - protein, 9 aa, synthetic construct
GGAGHDELH

SEQ ID NO: 21339 - protein, 9 aa, synthetic construct
GGAGHDFAS

SEQ ID NO: 21340 - protein, 9 aa, synthetic construct
GGFGADTIY

SEQ ID NO: 21341 - protein, 9 aa, synthetic construct
GGFGADTLF

SEQ ID NO: 21342 - protein, 9 aa, synthetic construct
GGFGADTLH

SEQ ID NO: 21343 - protein, 9 aa, synthetic construct
GGEGNDKAN

SEQ ID NO: 21344 - protein, 9 aa, synthetic construct
GGTGEDEIV

SEQ ID NO: 21345 - protein, 9 aa, synthetic construct
GGAGHDGLE

SEQ ID NO: 21346 - protein, 9 aa, synthetic construct
GGTGDDYYI

SEQ ID NO: 21347 - protein, 9 aa, synthetic construct
GGAGHDHFV

SEQ ID NO: 21348 - protein, 9 aa, synthetic construct
GGTGDDYVS

SEQ ID NO: 21349 - protein, 9 aa, synthetic construct
GGTGDDYVD

SEQ ID NO: 21350 - protein, 9 aa, synthetic construct
GGTGDDYMR

SEQ ID NO: 21351 - protein, 9 aa, synthetic construct
GGAGHDHIT

SEQ ID NO: 21352 - protein, 9 aa, synthetic construct
GGAGHDHIV

SEQ ID NO: 21353 - protein, 9 aa, synthetic construct
GGTGDDYLR

SEQ ID NO: 21354 - protein, 9 aa, synthetic construct
GGTGDDYLL

SEQ ID NO: 21355 - protein, 9 aa, synthetic construct
GGTGDDYLI

SEQ ID NO: 21356 - protein, 9 aa, synthetic construct
GGAGHDIAD

SEQ ID NO: 21357 - protein, 9 aa, synthetic construct
GGAGHDIAS

SEQ ID NO: 21358 - protein, 9 aa, synthetic construct
GGAGHDIFD

SEQ ID NO: 21359 - protein, 9 aa, synthetic construct
GGTGDDTVI

SEQ ID NO: 21360 - protein, 9 aa, synthetic construct
GGFGADVFA

SEQ ID NO: 21361 - protein, 9 aa, synthetic construct
GGAGHDKIL

SEQ ID NO: 21362 - protein, 9 aa, synthetic construct
GGTGDDTLW

SEQ ID NO: 21363 - protein, 9 aa, synthetic construct
GGTGDDRIY

SEQ ID NO: 21364 - protein, 9 aa, synthetic construct
GGTGDDRIT

SEQ ID NO: 21365 - protein, 9 aa, synthetic construct
GGTGDDRIL

SEQ ID NO: 21366 - protein, 9 aa, synthetic construct
GGTGDDRFL

SEQ ID NO: 21367 - protein, 9 aa, synthetic construct
GGAGHDLVD

SEQ ID NO: 21368 - protein, 9 aa, synthetic construct
GGTGDDQVI

SEQ ID NO: 21369 - protein, 9 aa, synthetic construct
GGTGDDQVE

SEQ ID NO: 21370 - protein, 9 aa, synthetic construct
GGTGDDQMA

SEQ ID NO: 21371 - protein, 9 aa, synthetic construct
GGTGDDQLN

SEQ ID NO: 21372 - protein, 9 aa, synthetic construct
GGTGDDQLA

SEQ ID NO: 21373 - protein, 9 aa, synthetic construct
GGTGDDQIY

SEQ ID NO: 21374 - protein, 9 aa, synthetic construct
GGFGDDALS

SEQ ID NO: 21375 - protein, 9 aa, synthetic construct
GGAGHDMIR

SEQ ID NO: 21376 - protein, 9 aa, synthetic construct
GGAGHDMLF

SEQ ID NO: 21377 - protein, 9 aa, synthetic construct
GGAGHDMLL

SEQ ID NO: 21378 - protein, 9 aa, synthetic construct
GGAGHDMLT

SEQ ID NO: 21379 - protein, 9 aa, synthetic construct
GGAGHDMLV

SEQ ID NO: 21380 - protein, 9 aa, synthetic construct
GGAGHDMLY

SEQ ID NO: 21381 - protein, 9 aa, synthetic construct
GGAGHDNIA

SEQ ID NO: 21382 - protein, 9 aa, synthetic construct
GGTGDDNLG

SEQ ID NO: 21383 - protein, 9 aa, synthetic construct
GGTGDDNIN

SEQ ID NO: 21384 - protein, 9 aa, synthetic construct
GGAGHDNLF

SEQ ID NO: 21385 - protein, 9 aa, synthetic construct
GGEGNDILG

SEQ ID NO: 21386 - protein, 9 aa, synthetic construct
GGTGDDMLW

SEQ ID NO: 21387 - protein, 9 aa, synthetic construct
GGAGHDNLT

SEQ ID NO: 21388 - protein, 9 aa, synthetic construct
GGTGDDRLT

SEQ ID NO: 21389 - protein, 9 aa, synthetic construct
GGTGDDRMF

SEQ ID NO: 21390 - protein, 9 aa, synthetic construct
GGTGDDRVI

SEQ ID NO: 21391 - protein, 9 aa, synthetic construct
GGAGHDLIA

SEQ ID NO: 21392 - protein, 9 aa, synthetic construct
GGFGADVIR

SEQ ID NO: 21393 - protein, 9 aa, synthetic construct
GGAGHDKLD

SEQ ID NO: 21394 - protein, 9 aa, synthetic construct
GGEGNDIMY

SEQ ID NO: 21395 - protein, 9 aa, synthetic construct
GGAGHDKLS

SEQ ID NO: 21396 - protein, 9 aa, synthetic construct
GGTGDDTAY

SEQ ID NO: 21397 - protein, 9 aa, synthetic construct
GGTGDDTAS

SEQ ID NO: 21398 - protein, 9 aa, synthetic construct
GGAGHDKMG

SEQ ID NO: 21399 - protein, 9 aa, synthetic construct
GGTGDDTAL

SEQ ID NO: 21400 - protein, 9 aa, synthetic construct
GGTGDDTAF

SEQ ID NO: 21401 - protein, 9 aa, synthetic construct
GGAGHDKVF

SEQ ID NO: 21402 - protein, 9 aa, synthetic construct
GGAGHDLAY

SEQ ID NO: 21403 - protein, 9 aa, synthetic construct
GGTGDDSVI

SEQ ID NO: 21404 - protein, 9 aa, synthetic construct
GGTGDDRVN

SEQ ID NO: 21405 - protein, 9 aa, synthetic construct
GGAGHDLIF

SEQ ID NO: 21406 - protein, 9 aa, synthetic construct
GGAGHDLIG

SEQ ID NO: 21407 - protein, 9 aa, synthetic construct
GGTGDDSMR

SEQ ID NO: 21408 - protein, 9 aa, synthetic construct
GGTGDDSLK

SEQ ID NO: 21409 - protein, 9 aa, synthetic construct
GGTGDDSIV

SEQ ID NO: 21410 - protein, 9 aa, synthetic construct
GGTGDDSII

SEQ ID NO: 21411 - protein, 9 aa, synthetic construct
GGTGDDSIF

SEQ ID NO: 21412 - protein, 9 aa, synthetic construct
GGTGDDSAD

SEQ ID NO: 21413 - protein, 9 aa, synthetic construct
GGTGDDRVY

SEQ ID NO: 21414 - protein, 9 aa, synthetic construct
GGTGDDRVS

SEQ ID NO: 21415 - protein, 9 aa, synthetic construct
GGTGDDRVQ

SEQ ID NO: 21416 - protein, 9 aa, synthetic construct
GGTGEDLLI

SEQ ID NO: 21417 - protein, 9 aa, synthetic construct
GGEGNDKIS

SEQ ID NO: 21418 - protein, 9 aa, synthetic construct
GGTGEDLLR

SEQ ID NO: 21419 - protein, 9 aa, synthetic construct
GGTGFDTIE

SEQ ID NO: 21420 - protein, 9 aa, synthetic construct
GGTGGDKLY

SEQ ID NO: 21421 - protein, 9 aa, synthetic construct
GGAGGDTMI

SEQ ID NO: 21422 - protein, 9 aa, synthetic construct
GGFGADLFV

SEQ ID NO: 21423 - protein, 9 aa, synthetic construct
GGTGGDILR

SEQ ID NO: 21424 - protein, 9 aa, synthetic construct
GGAGGDTVR

SEQ ID NO: 21425 - protein, 9 aa, synthetic construct
GGFGADLLR

SEQ ID NO: 21426 - protein, 9 aa, synthetic construct
GGTGGDFLW

SEQ ID NO: 21427 - protein, 9 aa, synthetic construct
GGAGGDTYN

SEQ ID NO: 21428 - protein, 9 aa, synthetic construct
GGAGGDTYR

SEQ ID NO: 21429 - protein, 9 aa, synthetic construct
GGFGADLMA

SEQ ID NO: 21430 - protein, 9 aa, synthetic construct
GGAGGDVFA

SEQ ID NO: 21431 - protein, 9 aa, synthetic construct
GGFGADMLE

SEQ ID NO: 21432 - protein, 9 aa, synthetic construct
GGAGGDVFI

SEQ ID NO: 21433 - protein, 9 aa, synthetic construct
GGFGADMLT

SEQ ID NO: 21434 - protein, 9 aa, synthetic construct
GGFGADNFL

SEQ ID NO: 21435 - protein, 9 aa, synthetic construct
GGTGGDALN

SEQ ID NO: 21436 - protein, 9 aa, synthetic construct
GGTGFDYMV

SEQ ID NO: 21437 - protein, 9 aa, synthetic construct
GGTGFDVVD

SEQ ID NO: 21438 - protein, 9 aa, synthetic construct
GGAGGDVIL

SEQ ID NO: 21439 - protein, 9 aa, synthetic construct
GGAGGDVIS

SEQ ID NO: 21440 - protein, 9 aa, synthetic construct
GGEGNDKLV

SEQ ID NO: 21441 - protein, 9 aa, synthetic construct
GGAGGDVLE

SEQ ID NO: 21442 - protein, 9 aa, synthetic construct
GGEGNDKLT

SEQ ID NO: 21443 - protein, 9 aa, synthetic construct
GGTGFDTLT

SEQ ID NO: 21444 - protein, 9 aa, synthetic construct
GGTGFDTLR

SEQ ID NO: 21445 - protein, 9 aa, synthetic construct
GGTGGDKMI

SEQ ID NO: 21446 - protein, 9 aa, synthetic construct
GGTGGDKMT

SEQ ID NO: 21447 - protein, 9 aa, synthetic construct
GGAGGDTMH

SEQ ID NO: 21448 - protein, 9 aa, synthetic construct
GGFGADIYI

SEQ ID NO: 21449 - protein, 9 aa, synthetic construct
GGTGGDTLR

SEQ ID NO: 21450 - protein, 9 aa, synthetic construct
GGAGGDTAS

SEQ ID NO: 21451 - protein, 9 aa, synthetic construct
GGEGNDLFI

SEQ ID NO: 21452 - protein, 9 aa, synthetic construct
GGTGGDTLE

SEQ ID NO: 21453 - protein, 9 aa, synthetic construct
GGAGGDTFR

SEQ ID NO: 21454 - protein, 9 aa, synthetic construct
GGTGGDTFL

SEQ ID NO: 21455 - protein, 9 aa, synthetic construct
GGFGADIMK

SEQ ID NO: 21456 - protein, 9 aa, synthetic construct
GGTGGDSLH

SEQ ID NO: 21457 - protein, 9 aa, synthetic construct
GGEGNDLAY

SEQ ID NO: 21458 - protein, 9 aa, synthetic construct
GGTGGDRVF

SEQ ID NO: 21459 - protein, 9 aa, synthetic construct
GGEGNDLAW

SEQ ID NO: 21460 - protein, 9 aa, synthetic construct
GGTGGDRLT

SEQ ID NO: 21461 - protein, 9 aa, synthetic construct
GGTGGDLLI

SEQ ID NO: 21462 - protein, 9 aa, synthetic construct
GGAGGDTIR

SEQ ID NO: 21463 - protein, 9 aa, synthetic construct
GGTGGDRLN

SEQ ID NO: 21464 - protein, 9 aa, synthetic construct
GGTGGDRFV

SEQ ID NO: 21465 - protein, 9 aa, synthetic construct
GGTGGDQMI

SEQ ID NO: 21466 - protein, 9 aa, synthetic construct
GGTGGDNMF

SEQ ID NO: 21467 - protein, 9 aa, synthetic construct
GGTGGDNLY

SEQ ID NO: 21468 - protein, 9 aa, synthetic construct
GGTGGDNLR

SEQ ID NO: 21469 - protein, 9 aa, synthetic construct
GGAGGDTLF

SEQ ID NO: 21470 - protein, 9 aa, synthetic construct
GGAGGDTLG

SEQ ID NO: 21471 - protein, 9 aa, synthetic construct
GGTGGDLYI

SEQ ID NO: 21472 - protein, 9 aa, synthetic construct
GGTGGDLMS

SEQ ID NO: 21473 - protein, 9 aa, synthetic construct
GGTGFDTIH

SEQ ID NO: 21474 - protein, 9 aa, synthetic construct
GGTGFDTFY

SEQ ID NO: 21475 - protein, 9 aa, synthetic construct
GGAGHDDLQ

SEQ ID NO: 21476 - protein, 9 aa, synthetic construct
GGTGFDTFV

SEQ ID NO: 21477 - protein, 9 aa, synthetic construct
GGTGEDVLN

SEQ ID NO: 21478 - protein, 9 aa, synthetic construct
GGTGEDVLE

SEQ ID NO: 21479 - protein, 9 aa, synthetic construct
GGTGEDTYY

SEQ ID NO: 21480 - protein, 9 aa, synthetic construct
GGFGADSLM

SEQ ID NO: 21481 - protein, 9 aa, synthetic construct
GGTGEDTMT

SEQ ID NO: 21482 - protein, 9 aa, synthetic construct
GGTGEDTMN

SEQ ID NO: 21483 - protein, 9 aa, synthetic construct
GGTGEDTLY

SEQ ID NO: 21484 - protein, 9 aa, synthetic construct
GGTGEDTLT

SEQ ID NO: 21485 - protein, 9 aa, synthetic construct
GGTGEDTLE

SEQ ID NO: 21486 - protein, 9 aa, synthetic construct
GGTGEDTIY

SEQ ID NO: 21487 - protein, 9 aa, synthetic construct
GGTGEDTIM

SEQ ID NO: 21488 - protein, 9 aa, synthetic construct
GGTGEDTID

SEQ ID NO: 21489 - protein, 9 aa, synthetic construct
GGAGHDAFV

SEQ ID NO: 21490 - protein, 9 aa, synthetic construct
GGTGEDSMN

SEQ ID NO: 21491 - protein, 9 aa, synthetic construct
GGTGEDSLL

SEQ ID NO: 21492 - protein, 9 aa, synthetic construct
GGFGADSVI

SEQ ID NO: 21493 - protein, 9 aa, synthetic construct
GGTGEDRVF

SEQ ID NO: 21494 - protein, 9 aa, synthetic construct
GGAGHDALI

SEQ ID NO: 21495 - protein, 9 aa, synthetic construct
GGAGHDALR

SEQ ID NO: 21496 - protein, 9 aa, synthetic construct
GGAGHDALV

SEQ ID NO: 21497 - protein, 9 aa, synthetic construct
GGTGEDQVT

SEQ ID NO: 21498 - protein, 9 aa, synthetic construct
GGFGADTFI

SEQ ID NO: 21499 - protein, 9 aa, synthetic construct
GGTGEDQIG

SEQ ID NO: 21500 - protein, 9 aa, synthetic construct
GGTGEDNIS

SEQ ID NO: 21501 - protein, 9 aa, synthetic construct
GGAGHDDIH

SEQ ID NO: 21502 - protein, 9 aa, synthetic construct
GGTGEDVLS

SEQ ID NO: 21503 - protein, 9 aa, synthetic construct
GGFGADSLI

SEQ ID NO: 21504 - protein, 9 aa, synthetic construct
GGAGGDWVV

SEQ ID NO: 21505 - protein, 9 aa, synthetic construct
GGTGFDMAD

SEQ ID NO: 21506 - protein, 9 aa, synthetic construct
GGTGFDTAR

SEQ ID NO: 21507 - protein, 9 aa, synthetic construct
GGAGGDVMD

SEQ ID NO: 21508 - protein, 9 aa, synthetic construct
GGTGFDSIL

SEQ ID NO: 21509 - protein, 9 aa, synthetic construct
GGTGFDSAD

SEQ ID NO: 21510 - protein, 9 aa, synthetic construct
GGTGFDRMS

SEQ ID NO: 21511 - protein, 9 aa, synthetic construct
GGAGGDVMK

SEQ ID NO: 21512 - protein, 9 aa, synthetic construct
GGTGFDRLF

SEQ ID NO: 21513 - protein, 9 aa, synthetic construct
GGFGADRFF

SEQ ID NO: 21514 - protein, 9 aa, synthetic construct
GGAGGDVMN

SEQ ID NO: 21515 - protein, 9 aa, synthetic construct
GGFGADRFG

SEQ ID NO: 21516 - protein, 9 aa, synthetic construct
GGAGGDVMT

SEQ ID NO: 21517 - protein, 9 aa, synthetic construct
GGAGGDVYV

SEQ ID NO: 21518 - protein, 9 aa, synthetic construct
GGTGFDAAS

SEQ ID NO: 21519 - protein, 9 aa, synthetic construct
GGFGADRLD

SEQ ID NO: 21520 - protein, 9 aa, synthetic construct
GGTGFDHLM

SEQ ID NO: 21521 - protein, 9 aa, synthetic construct
GGFGADRLS

SEQ ID NO: 21522 - protein, 9 aa, synthetic construct
GGTGFDFLT

SEQ ID NO: 21523 - protein, 9 aa, synthetic construct
GGTGFDFLS

SEQ ID NO: 21524 - protein, 9 aa, synthetic construct
GGAGGDWLL

SEQ ID NO: 21525 - protein, 9 aa, synthetic construct
GGFGADRLT

SEQ ID NO: 21526 - protein, 9 aa, synthetic construct
GGFGADRME

SEQ ID NO: 21527 - protein, 9 aa, synthetic construct
GGTGFDEIH

SEQ ID NO: 21528 - protein, 9 aa, synthetic construct
GGAGGDWLT

SEQ ID NO: 21529 - protein, 9 aa, synthetic construct
GGTGFDAMF

SEQ ID NO: 21530 - protein, 9 aa, synthetic construct
GGTGDDMLI

SEQ ID NO: 21531 - protein, 9 aa, synthetic construct
GGFGDDDLQ

SEQ ID NO: 21532 - protein, 9 aa, synthetic construct
GGAGHDQIF

SEQ ID NO: 21533 - protein, 9 aa, synthetic construct
GGTGADRAW

SEQ ID NO: 21534 - protein, 9 aa, synthetic construct
GGAGHDYLD

SEQ ID NO: 21535 - protein, 9 aa, synthetic construct
GGTGADSLK

SEQ ID NO: 21536 - protein, 9 aa, synthetic construct
GGTGADSLH

SEQ ID NO: 21537 - protein, 9 aa, synthetic construct
GGAGHDYLI

SEQ ID NO: 21538 - protein, 9 aa, synthetic construct
GGTGADSIY

SEQ ID NO: 21539 - protein, 9 aa, synthetic construct
GGTGADSIT

SEQ ID NO: 21540 - protein, 9 aa, synthetic construct
GGTGADSIN

SEQ ID NO: 21541 - protein, 9 aa, synthetic construct
GGTGADSIL

SEQ ID NO: 21542 - protein, 9 aa, synthetic construct
GGAGHDYLY

SEQ ID NO: 21543 - protein, 9 aa, synthetic construct
GGTGADSIF

SEQ ID NO: 21544 - protein, 9 aa, synthetic construct
GGEGNDHLL

SEQ ID NO: 21545 - protein, 9 aa, synthetic construct
GGTGADSFT

SEQ ID NO: 21546 - protein, 9 aa, synthetic construct
GGAGIDAAD

SEQ ID NO: 21547 - protein, 9 aa, synthetic construct
GGAGIDAAS

SEQ ID NO: 21548 - protein, 9 aa, synthetic construct
GGFGDDLLI

SEQ ID NO: 21549 - protein, 9 aa, synthetic construct
GGTGADRVD

SEQ ID NO: 21550 - protein, 9 aa, synthetic construct
GGAGIDALD

SEQ ID NO: 21551 - protein, 9 aa, synthetic construct
GGAGIDALF

SEQ ID NO: 21552 - protein, 9 aa, synthetic construct
GGTGADRMF

SEQ ID NO: 21553 - protein, 9 aa, synthetic construct
GGAGIDALT

SEQ ID NO: 21554 - protein, 9 aa, synthetic construct
GGTGADRIT

SEQ ID NO: 21555 - protein, 9 aa, synthetic construct
GGAGIDALY

SEQ ID NO: 21556 - protein, 9 aa, synthetic construct
GGTGADRID

SEQ ID NO: 21557 - protein, 9 aa, synthetic construct
GGTGADRIA

SEQ ID NO: 21558 - protein, 9 aa, synthetic construct
GGEGNDHIY

SEQ ID NO: 21559 - protein, 9 aa, synthetic construct
GGAGHDWLR

SEQ ID NO: 21560 - protein, 9 aa, synthetic construct
GGEGNDHLR

SEQ ID NO: 21561 - protein, 9 aa, synthetic construct
GGTGADSVD

SEQ ID NO: 21562 - protein, 9 aa, synthetic construct
GGTGADTVF

SEQ ID NO: 21563 - protein, 9 aa, synthetic construct
GGTGADVIA

SEQ ID NO: 21564 - protein, 9 aa, synthetic construct
GGTGADVFY

SEQ ID NO: 21565 - protein, 9 aa, synthetic construct
GGAGHDVLT

SEQ ID NO: 21566 - protein, 9 aa, synthetic construct
GGTGADVFK

SEQ ID NO: 21567 - protein, 9 aa, synthetic construct
GGAGHDVLV

SEQ ID NO: 21568 - protein, 9 aa, synthetic construct
GGTGADTYQ

SEQ ID NO: 21569 - protein, 9 aa, synthetic construct
GGTGADTYK

SEQ ID NO: 21570 - protein, 9 aa, synthetic construct
GGEGNDHVF

SEQ ID NO: 21571 - protein, 9 aa, synthetic construct
GGAGHDVMH

SEQ ID NO: 21572 - protein, 9 aa, synthetic construct
GGAGHDVYI

SEQ ID NO: 21573 - protein, 9 aa, synthetic construct
GGAGHDVYN

SEQ ID NO: 21574 - protein, 9 aa, synthetic construct
GGTGADTLK

SEQ ID NO: 21575 - protein, 9 aa, synthetic construct
GGFGDDLIR

SEQ ID NO: 21576 - protein, 9 aa, synthetic construct
GGTGADTIV

SEQ ID NO: 21577 - protein, 9 aa, synthetic construct
GGTGADTIM

SEQ ID NO: 21578 - protein, 9 aa, synthetic construct
GGTGADTIK

SEQ ID NO: 21579 - protein, 9 aa, synthetic construct
GGTGADTIA

SEQ ID NO: 21580 - protein, 9 aa, synthetic construct
GGTGADTFY

SEQ ID NO: 21581 - protein, 9 aa, synthetic construct
GGTGADTFS

SEQ ID NO: 21582 - protein, 9 aa, synthetic construct
GGAGHDWIM

SEQ ID NO: 21583 - protein, 9 aa, synthetic construct
GGFGDDLIF

SEQ ID NO: 21584 - protein, 9 aa, synthetic construct
GGFGDDLIG

SEQ ID NO: 21585 - protein, 9 aa, synthetic construct
GGTGADTAF

SEQ ID NO: 21586 - protein, 9 aa, synthetic construct
GGTGADSYV

SEQ ID NO: 21587 - protein, 9 aa, synthetic construct
GGAGIDDID

SEQ ID NO: 21588 - protein, 9 aa, synthetic construct
GGTGADQYF

SEQ ID NO: 21589 - protein, 9 aa, synthetic construct
GGAGHDVLM

SEQ ID NO: 21590 - protein, 9 aa, synthetic construct
GGTGADQVN

SEQ ID NO: 21591 - protein, 9 aa, synthetic construct
GGFGDDRLN

SEQ ID NO: 21592 - protein, 9 aa, synthetic construct
GGEGNDGIN

SEQ ID NO: 21593 - protein, 9 aa, synthetic construct
GGEGNDFYV

SEQ ID NO: 21594 - protein, 9 aa, synthetic construct
GGTGADLVA

SEQ ID NO: 21595 - protein, 9 aa, synthetic construct
GGTGADLMY

SEQ ID NO: 21596 - protein, 9 aa, synthetic construct
GGEGNDFVS

SEQ ID NO: 21597 - protein, 9 aa, synthetic construct
GGTGADLML

SEQ ID NO: 21598 - protein, 9 aa, synthetic construct
GGTGADLLS

SEQ ID NO: 21599 - protein, 9 aa, synthetic construct
GGTGADLLM

SEQ ID NO: 21600 - protein, 9 aa, synthetic construct
GGTGADKMY

SEQ ID NO: 21601 - protein, 9 aa, synthetic construct
GGTGADKMI

SEQ ID NO: 21602 - protein, 9 aa, synthetic construct
GGTGADKLV

SEQ ID NO: 21603 - protein, 9 aa, synthetic construct
GGTGADKLQ

SEQ ID NO: 21604 - protein, 9 aa, synthetic construct
GGAGIDIMT

SEQ ID NO: 21605 - protein, 9 aa, synthetic construct
GGAGIDIVR

SEQ ID NO: 21606 - protein, 9 aa, synthetic construct
GGAGIDKLH

SEQ ID NO: 21607 - protein, 9 aa, synthetic construct
GGTGADIVL

SEQ ID NO: 21608 - protein, 9 aa, synthetic construct
GGTGADIMS

SEQ ID NO: 21609 - protein, 9 aa, synthetic construct
GGTGADIME

SEQ ID NO: 21610 - protein, 9 aa, synthetic construct
GGTGADILV

SEQ ID NO: 21611 - protein, 9 aa, synthetic construct
GGTGADILR

SEQ ID NO: 21612 - protein, 9 aa, synthetic construct
GGTGADILD

SEQ ID NO: 21613 - protein, 9 aa, synthetic construct
GGEGNDFLT

SEQ ID NO: 21614 - protein, 9 aa, synthetic construct
GGTGADIFA

SEQ ID NO: 21615 - protein, 9 aa, synthetic construct
GGEGNDFLR

SEQ ID NO: 21616 - protein, 9 aa, synthetic construct
GGAGIDIFI

SEQ ID NO: 21617 - protein, 9 aa, synthetic construct
GGTGADMIF

SEQ ID NO: 21618 - protein, 9 aa, synthetic construct
GGTGADMLD

SEQ ID NO: 21619 - protein, 9 aa, synthetic construct
GGTGADQFH

SEQ ID NO: 21620 - protein, 9 aa, synthetic construct
GGTGADQMY

SEQ ID NO: 21621 - protein, 9 aa, synthetic construct
GGAGIDDIQ

SEQ ID NO: 21622 - protein, 9 aa, synthetic construct
GGTGADQMK

SEQ ID NO: 21623 - protein, 9 aa, synthetic construct
GGAGIDDVF

SEQ ID NO: 21624 - protein, 9 aa, synthetic construct
GGAGIDDVY

SEQ ID NO: 21625 - protein, 9 aa, synthetic construct
GGEGNDHID

SEQ ID NO: 21626 - protein, 9 aa, synthetic construct
GGAGIDEAR

SEQ ID NO: 21627 - protein, 9 aa, synthetic construct
GGTGADQLE

SEQ ID NO: 21628 - protein, 9 aa, synthetic construct
GGEGNDGLY

SEQ ID NO: 21629 - protein, 9 aa, synthetic construct
GGTGADQIV

SEQ ID NO: 21630 - protein, 9 aa, synthetic construct
GGTGADQFK

SEQ ID NO: 21631 - protein, 9 aa, synthetic construct
GGFGDDQIN

SEQ ID NO: 21632 - protein, 9 aa, synthetic construct
GGTGADMLI

SEQ ID NO: 21633 - protein, 9 aa, synthetic construct
GGAGIDFIY

SEQ ID NO: 21634 - protein, 9 aa, synthetic construct
GGEGNDGLL

SEQ ID NO: 21635 - protein, 9 aa, synthetic construct
GGEGNDGLF

SEQ ID NO: 21636 - protein, 9 aa, synthetic construct
GGTGADNLV

SEQ ID NO: 21637 - protein, 9 aa, synthetic construct
GGTGADNLR

SEQ ID NO: 21638 - protein, 9 aa, synthetic construct
GGTGADNLL

SEQ ID NO: 21639 - protein, 9 aa, synthetic construct
GGFGDDQLY

SEQ ID NO: 21640 - protein, 9 aa, synthetic construct
GGAGIDFVY

SEQ ID NO: 21641 - protein, 9 aa, synthetic construct
GGAGIDGLR

SEQ ID NO: 21642 - protein, 9 aa, synthetic construct
GGEGNDGIS

SEQ ID NO: 21643 - protein, 9 aa, synthetic construct
GGTGADMLT

SEQ ID NO: 21644 - protein, 9 aa, synthetic construct
GGTGADVIF

SEQ ID NO: 21645 - protein, 9 aa, synthetic construct
GGTGADVLE

SEQ ID NO: 21646 - protein, 9 aa, synthetic construct
GGFGDDDLT

SEQ ID NO: 21647 - protein, 9 aa, synthetic construct
GGAGHDTFL

SEQ ID NO: 21648 - protein, 9 aa, synthetic construct
GGTGDDIIR

SEQ ID NO: 21649 - protein, 9 aa, synthetic construct
GGTGDDIIL

SEQ ID NO: 21650 - protein, 9 aa, synthetic construct
GGTGDDIIA

SEQ ID NO: 21651 - protein, 9 aa, synthetic construct
GGTGDDIFD

SEQ ID NO: 21652 - protein, 9 aa, synthetic construct
GGTGDDIAR

SEQ ID NO: 21653 - protein, 9 aa, synthetic construct
GGTGDDHVF

SEQ ID NO: 21654 - protein, 9 aa, synthetic construct
GGTGDDHLY

SEQ ID NO: 21655 - protein, 9 aa, synthetic construct
GGAGHDSLA

SEQ ID NO: 21656 - protein, 9 aa, synthetic construct
GGTGDDHIV

SEQ ID NO: 21657 - protein, 9 aa, synthetic construct
GGTGDDHIE

SEQ ID NO: 21658 - protein, 9 aa, synthetic construct
GGTGDDGLT

SEQ ID NO: 21659 - protein, 9 aa, synthetic construct
GGTGDDFYV

SEQ ID NO: 21660 - protein, 9 aa, synthetic construct
GGFGDDHVA

SEQ ID NO: 21661 - protein, 9 aa, synthetic construct
GGTGDDFYL

SEQ ID NO: 21662 - protein, 9 aa, synthetic construct
GGTGDDFVY

SEQ ID NO: 21663 - protein, 9 aa, synthetic construct
GGAGHDTAD

SEQ ID NO: 21664 - protein, 9 aa, synthetic construct
GGAGHDTAF

SEQ ID NO: 21665 - protein, 9 aa, synthetic construct
GGTGDDFVD

SEQ ID NO: 21666 - protein, 9 aa, synthetic construct
GGTGDDFMA

SEQ ID NO: 21667 - protein, 9 aa, synthetic construct
GGTGDDFLT

SEQ ID NO: 21668 - protein, 9 aa, synthetic construct
GGAGHDTAV

SEQ ID NO: 21669 - protein, 9 aa, synthetic construct
GGTGDDFLN

SEQ ID NO: 21670 - protein, 9 aa, synthetic construct
GGTGDDFLL

SEQ ID NO: 21671 - protein, 9 aa, synthetic construct
GGTGDDFLA

SEQ ID NO: 21672 - protein, 9 aa, synthetic construct
GGEGNDIFA

SEQ ID NO: 21673 - protein, 9 aa, synthetic construct
GGTGDDILH

SEQ ID NO: 21674 - protein, 9 aa, synthetic construct
GGTGDDILM

SEQ ID NO: 21675 - protein, 9 aa, synthetic construct
GGTGDDILQ

SEQ ID NO: 21676 - protein, 9 aa, synthetic construct
GGTGDDLAY

SEQ ID NO: 21677 - protein, 9 aa, synthetic construct
GGTGDDLYR

SEQ ID NO: 21678 - protein, 9 aa, synthetic construct
GGTGDDLYF

SEQ ID NO: 21679 - protein, 9 aa, synthetic construct
GGTGDDLYD

SEQ ID NO: 21680 - protein, 9 aa, synthetic construct
GGFGDDEIT

SEQ ID NO: 21681 - protein, 9 aa, synthetic construct
GGTGDDLVL

SEQ ID NO: 21682 - protein, 9 aa, synthetic construct
GGTGDDLVE

SEQ ID NO: 21683 - protein, 9 aa, synthetic construct
GGTGDDLMD

SEQ ID NO: 21684 - protein, 9 aa, synthetic construct
GGAGHDRIE

SEQ ID NO: 21685 - protein, 9 aa, synthetic construct
GGTGDDLIM

SEQ ID NO: 21686 - protein, 9 aa, synthetic construct
GGAGHDRIR

SEQ ID NO: 21687 - protein, 9 aa, synthetic construct
GGTGDDLFL

SEQ ID NO: 21688 - protein, 9 aa, synthetic construct
GGEGNDIIR

SEQ ID NO: 21689 - protein, 9 aa, synthetic construct
GGEGNDIIL

SEQ ID NO: 21690 - protein, 9 aa, synthetic construct
GGAGHDRIY

SEQ ID NO: 21691 - protein, 9 aa, synthetic construct
GGTGDDKVY

SEQ ID NO: 21692 - protein, 9 aa, synthetic construct
GGTGDDKLS

SEQ ID NO: 21693 - protein, 9 aa, synthetic construct
GGTGDDKLN

SEQ ID NO: 21694 - protein, 9 aa, synthetic construct
GGTGDDIYW

SEQ ID NO: 21695 - protein, 9 aa, synthetic construct
GGAGHDRVF

SEQ ID NO: 21696 - protein, 9 aa, synthetic construct
GGTGDDIVQ

SEQ ID NO: 21697 - protein, 9 aa, synthetic construct
GGAGHDSFE

SEQ ID NO: 21698 - protein, 9 aa, synthetic construct
GGTGDDIVE

SEQ ID NO: 21699 - protein, 9 aa, synthetic construct
GGTGDDIMT

SEQ ID NO: 21700 - protein, 9 aa, synthetic construct
GGTGDDIML

SEQ ID NO: 21701 - protein, 9 aa, synthetic construct
GGTGDDFIV

SEQ ID NO: 21702 - protein, 9 aa, synthetic construct
GGTGDDFIQ

SEQ ID NO: 21703 - protein, 9 aa, synthetic construct
GGTGADVLH

SEQ ID NO: 21704 - protein, 9 aa, synthetic construct
GGTGDDFIN

SEQ ID NO: 21705 - protein, 9 aa, synthetic construct
GGFGDDILT

SEQ ID NO: 21706 - protein, 9 aa, synthetic construct
GGTGDDALG

SEQ ID NO: 21707 - protein, 9 aa, synthetic construct
GGTGDDALF

SEQ ID NO: 21708 - protein, 9 aa, synthetic construct
GGEGNDIAR

SEQ ID NO: 21709 - protein, 9 aa, synthetic construct
GGAGHDTML

SEQ ID NO: 21710 - protein, 9 aa, synthetic construct
GGTGDDAFY

SEQ ID NO: 21711 - protein, 9 aa, synthetic construct
GGTGCDRLV

SEQ ID NO: 21712 - protein, 9 aa, synthetic construct
GGFGDDKIG

SEQ ID NO: 21713 - protein, 9 aa, synthetic construct
GGFGDDKIL

SEQ ID NO: 21714 - protein, 9 aa, synthetic construct
GGTGADYMA

SEQ ID NO: 21715 - protein, 9 aa, synthetic construct
GGTGADYLS

SEQ ID NO: 21716 - protein, 9 aa, synthetic construct
GGTGADYLQ

SEQ ID NO: 21717 - protein, 9 aa, synthetic construct
GGTGADYLG

SEQ ID NO: 21718 - protein, 9 aa, synthetic construct
GGTGADYLE

SEQ ID NO: 21719 - protein, 9 aa, synthetic construct
GGTGADYLA

SEQ ID NO: 21720 - protein, 9 aa, synthetic construct
GGAGHDVFV

SEQ ID NO: 21721 - protein, 9 aa, synthetic construct
GGTGADYFV

SEQ ID NO: 21722 - protein, 9 aa, synthetic construct
GGTGADYFI

SEQ ID NO: 21723 - protein, 9 aa, synthetic construct
GGFGDDKLS

SEQ ID NO: 21724 - protein, 9 aa, synthetic construct
GGAGHDVIS

SEQ ID NO: 21725 - protein, 9 aa, synthetic construct
GGAGHDVIY

SEQ ID NO: 21726 - protein, 9 aa, synthetic construct
GGTGADVYK

SEQ ID NO: 21727 - protein, 9 aa, synthetic construct
GGTGADVVY

SEQ ID NO: 21728 - protein, 9 aa, synthetic construct
GGTGADVMN

SEQ ID NO: 21729 - protein, 9 aa, synthetic construct
GGTGADVMD

SEQ ID NO: 21730 - protein, 9 aa, synthetic construct
GGTGDDALK

SEQ ID NO: 21731 - protein, 9 aa, synthetic construct
GGTGDDALL

SEQ ID NO: 21732 - protein, 9 aa, synthetic construct
GGTGDDALQ

SEQ ID NO: 21733 - protein, 9 aa, synthetic construct
GGTGDDEIV

SEQ ID NO: 21734 - protein, 9 aa, synthetic construct
GGTGDDFII

SEQ ID NO: 21735 - protein, 9 aa, synthetic construct
GGFGDDIIR

SEQ ID NO: 21736 - protein, 9 aa, synthetic construct
GGFGDDILA

SEQ ID NO: 21737 - protein, 9 aa, synthetic construct
GGTGDDEMF

SEQ ID NO: 21738 - protein, 9 aa, synthetic construct
GGAGHDTIH

SEQ ID NO: 21739 - protein, 9 aa, synthetic construct
GGTGDDELQ

SEQ ID NO: 21740 - protein, 9 aa, synthetic construct
GGTGDDELN

SEQ ID NO: 21741 - protein, 9 aa, synthetic construct
GGFGDDILE

SEQ ID NO: 21742 - protein, 9 aa, synthetic construct
GGTGDDELI

SEQ ID NO: 21743 - protein, 9 aa, synthetic construct
GGTGDDELF

SEQ ID NO: 21744 - protein, 9 aa, synthetic construct
GGAGHDTIS

SEQ ID NO: 21745 - protein, 9 aa, synthetic construct
GGTGDDEII

SEQ ID NO: 21746 - protein, 9 aa, synthetic construct
GGTGDDAYY

SEQ ID NO: 21747 - protein, 9 aa, synthetic construct
GGTGDDEFV

SEQ ID NO: 21748 - protein, 9 aa, synthetic construct
GGTGDDDYI

SEQ ID NO: 21749 - protein, 9 aa, synthetic construct
GGTGDDDMF

SEQ ID NO: 21750 - protein, 9 aa, synthetic construct
GGTGDDDMD

SEQ ID NO: 21751 - protein, 9 aa, synthetic construct
GGAGHDTLG

SEQ ID NO: 21752 - protein, 9 aa, synthetic construct
GGTGDDDLE

SEQ ID NO: 21753 - protein, 9 aa, synthetic construct
GGTGDDDLD

SEQ ID NO: 21754 - protein, 9 aa, synthetic construct
GGTGDDDIS

SEQ ID NO: 21755 - protein, 9 aa, synthetic construct
GGAGHDTLK

SEQ ID NO: 21756 - protein, 9 aa, synthetic construct
GGEGNDIAY

SEQ ID NO: 21757 - protein, 9 aa, synthetic construct
GGTGDDDID

SEQ ID NO: 21758 - protein, 9 aa, synthetic construct
GGAGLDALF

SEQ ID NO: 21759 - protein, 9 aa, synthetic construct
GGAGLDALI

SEQ ID NO: 21760 - protein, 9 aa, synthetic construct
GGAGLDALN

SEQ ID NO: 21761 - protein, 9 aa, synthetic construct
GGAGNDLYW

SEQ ID NO: 21762 - protein, 9 aa, synthetic construct
GGAGNDMFD

SEQ ID NO: 21763 - protein, 9 aa, synthetic construct
GGSGEDYLD

SEQ ID NO: 21764 - protein, 9 aa, synthetic construct
GGSGEDVLV

SEQ ID NO: 21765 - protein, 9 aa, synthetic construct
GGSGEDVLT

SEQ ID NO: 21766 - protein, 9 aa, synthetic construct
GGSGEDVLR

SEQ ID NO: 21767 - protein, 9 aa, synthetic construct
GGFGRDTLI

SEQ ID NO: 21768 - protein, 9 aa, synthetic construct
GGSGEDVLD

SEQ ID NO: 21769 - protein, 9 aa, synthetic construct
GGSGEDVFR

SEQ ID NO: 21770 - protein, 9 aa, synthetic construct
GGAGNDMIS

SEQ ID NO: 21771 - protein, 9 aa, synthetic construct
GGAGNDMIT

SEQ ID NO: 21772 - protein, 9 aa, synthetic construct
GGSGEDTLT

SEQ ID NO: 21773 - protein, 9 aa, synthetic construct
GGFGRDTLN

SEQ ID NO: 21774 - protein, 9 aa, synthetic construct
GGAGNDMIW

SEQ ID NO: 21775 - protein, 9 aa, synthetic construct
GGSGEDTIS

SEQ ID NO: 21776 - protein, 9 aa, synthetic construct
GGAGNDMLE

SEQ ID NO: 21777 - protein, 9 aa, synthetic construct
GGSGEDTIF

SEQ ID NO: 21778 - protein, 9 aa, synthetic construct
GGSGEDTAE

SEQ ID NO: 21779 - protein, 9 aa, synthetic construct
GGSGEDSMS

SEQ ID NO: 21780 - protein, 9 aa, synthetic construct
GGSGEDSMF

SEQ ID NO: 21781 - protein, 9 aa, synthetic construct
GGSGEDSLS

SEQ ID NO: 21782 - protein, 9 aa, synthetic construct
GGSGEDSLF

SEQ ID NO: 21783 - protein, 9 aa, synthetic construct
GGEGIDTMA

SEQ ID NO: 21784 - protein, 9 aa, synthetic construct
GGAGNDMMN

SEQ ID NO: 21785 - protein, 9 aa, synthetic construct
GGSGEDRMS

SEQ ID NO: 21786 - protein, 9 aa, synthetic construct
GGSGEDRLS

SEQ ID NO: 21787 - protein, 9 aa, synthetic construct
GGAGNDMAV

SEQ ID NO: 21788 - protein, 9 aa, synthetic construct
GGSGFDFAR

SEQ ID NO: 21789 - protein, 9 aa, synthetic construct
GGEGLDTVL

SEQ ID NO: 21790 - protein, 9 aa, synthetic construct
GGSGFDILT

SEQ ID NO: 21791 - protein, 9 aa, synthetic construct
GGSGGDALN

SEQ ID NO: 21792 - protein, 9 aa, synthetic construct
GGSGGDALI

SEQ ID NO: 21793 - protein, 9 aa, synthetic construct
GGAGNDLIW

SEQ ID NO: 21794 - protein, 9 aa, synthetic construct
GGSGGDAAS

SEQ ID NO: 21795 - protein, 9 aa, synthetic construct
GGSGFDYMV

SEQ ID NO: 21796 - protein, 9 aa, synthetic construct
GGSGFDYAD

SEQ ID NO: 21797 - protein, 9 aa, synthetic construct
GGSGFDWLF

SEQ ID NO: 21798 - protein, 9 aa, synthetic construct
GGSGFDVVE

SEQ ID NO: 21799 - protein, 9 aa, synthetic construct
GGSGFDTVV

SEQ ID NO: 21800 - protein, 9 aa, synthetic construct
GGSGFDTVS

SEQ ID NO: 21801 - protein, 9 aa, synthetic construct
GGSGFDTVD

SEQ ID NO: 21802 - protein, 9 aa, synthetic construct
GGSGFDTLS

SEQ ID NO: 21803 - protein, 9 aa, synthetic construct
GGSGFDTIT

SEQ ID NO: 21804 - protein, 9 aa, synthetic construct
GGSGFDTFD

SEQ ID NO: 21805 - protein, 9 aa, synthetic construct
GGSGFDTAV

SEQ ID NO: 21806 - protein, 9 aa, synthetic construct
GGSGFDSVS

SEQ ID NO: 21807 - protein, 9 aa, synthetic construct
GGSGFDSVE

SEQ ID NO: 21808 - protein, 9 aa, synthetic construct
GGSGFDSIN

SEQ ID NO: 21809 - protein, 9 aa, synthetic construct
GGFGRDSAS

SEQ ID NO: 21810 - protein, 9 aa, synthetic construct
GGSGFDNLD

SEQ ID NO: 21811 - protein, 9 aa, synthetic construct
GGSGFDMLN

SEQ ID NO: 21812 - protein, 9 aa, synthetic construct
GGSGFDLLN

SEQ ID NO: 21813 - protein, 9 aa, synthetic construct
GGSGFDKIF

SEQ ID NO: 21814 - protein, 9 aa, synthetic construct
GGAGNDLYF

SEQ ID NO: 21815 - protein, 9 aa, synthetic construct
GGSGFDILV

SEQ ID NO: 21816 - protein, 9 aa, synthetic construct
GGSGEDRLF

SEQ ID NO: 21817 - protein, 9 aa, synthetic construct
GGEGIDTLR

SEQ ID NO: 21818 - protein, 9 aa, synthetic construct
GGSGEDRIQ

SEQ ID NO: 21819 - protein, 9 aa, synthetic construct
GGSGEDMLD

SEQ ID NO: 21820 - protein, 9 aa, synthetic construct
GGAGNDNMT

SEQ ID NO: 21821 - protein, 9 aa, synthetic construct
GGMGADRLV

SEQ ID NO: 21822 - protein, 9 aa, synthetic construct
GGSGDDYLL

SEQ ID NO: 21823 - protein, 9 aa, synthetic construct
GGSGDDYLG

SEQ ID NO: 21824 - protein, 9 aa, synthetic construct
GGSGDDYLE

SEQ ID NO: 21825 - protein, 9 aa, synthetic construct
GGSGDDYLA

SEQ ID NO: 21826 - protein, 9 aa, synthetic construct
GGAGNDNVS

SEQ ID NO: 21827 - protein, 9 aa, synthetic construct
GGAGNDNVV

SEQ ID NO: 21828 - protein, 9 aa, synthetic construct
GGSGDDYIF

SEQ ID NO: 21829 - protein, 9 aa, synthetic construct
GGSGDDYID

SEQ ID NO: 21830 - protein, 9 aa, synthetic construct
GGFGSDIFF

SEQ ID NO: 21831 - protein, 9 aa, synthetic construct
GGFGSDIIF

SEQ ID NO: 21832 - protein, 9 aa, synthetic construct
GGAGNDQAY

SEQ ID NO: 21833 - protein, 9 aa, synthetic construct
GGAGNDQFG

SEQ ID NO: 21834 - protein, 9 aa, synthetic construct
GGAGNDQFI

SEQ ID NO: 21835 - protein, 9 aa, synthetic construct
GGSGDDWLV

SEQ ID NO: 21836 - protein, 9 aa, synthetic construct
GGSGDDWLT

SEQ ID NO: 21837 - protein, 9 aa, synthetic construct
GGAGNDQFL

SEQ ID NO: 21838 - protein, 9 aa, synthetic construct
GGSGDDWLD

SEQ ID NO: 21839 - protein, 9 aa, synthetic construct
GGEGIDTAI

SEQ ID NO: 21840 - protein, 9 aa, synthetic construct
GGSGDDWID

SEQ ID NO: 21841 - protein, 9 aa, synthetic construct
GGSGDDWFS

SEQ ID NO: 21842 - protein, 9 aa, synthetic construct
GGSGDDWFD

SEQ ID NO: 21843 - protein, 9 aa, synthetic construct
GGSGDDVYY

SEQ ID NO: 21844 - protein, 9 aa, synthetic construct
GGAGNDQIG

SEQ ID NO: 21845 - protein, 9 aa, synthetic construct
GGSGDDYLV

SEQ ID NO: 21846 - protein, 9 aa, synthetic construct
GGAGNDNMQ

SEQ ID NO: 21847 - protein, 9 aa, synthetic construct
GGSGDDYMG

SEQ ID NO: 21848 - protein, 9 aa, synthetic construct
GGAGNDNIT

SEQ ID NO: 21849 - protein, 9 aa, synthetic construct
GGAGNDNIF

SEQ ID NO: 21850 - protein, 9 aa, synthetic construct
GGSGEDLLT

SEQ ID NO: 21851 - protein, 9 aa, synthetic construct
GGSGEDLLI

SEQ ID NO: 21852 - protein, 9 aa, synthetic construct
GGSGEDLLF

SEQ ID NO: 21853 - protein, 9 aa, synthetic construct
GGSGEDLIY

SEQ ID NO: 21854 - protein, 9 aa, synthetic construct
GGSGEDLFL

SEQ ID NO: 21855 - protein, 9 aa, synthetic construct
GGFGSDDLT

SEQ ID NO: 21856 - protein, 9 aa, synthetic construct
GGSGEDKLR

SEQ ID NO: 21857 - protein, 9 aa, synthetic construct
GGAGNDNIN

SEQ ID NO: 21858 - protein, 9 aa, synthetic construct
GGAGNDNIQ

SEQ ID NO: 21859 - protein, 9 aa, synthetic construct
GGSGEDIMY

SEQ ID NO: 21860 - protein, 9 aa, synthetic construct
GGSGEDILF

SEQ ID NO: 21861 - protein, 9 aa, synthetic construct
GGSGDDYMV

SEQ ID NO: 21862 - protein, 9 aa, synthetic construct
GGSGEDILD

SEQ ID NO: 21863 - protein, 9 aa, synthetic construct
GGSGEDIFK

SEQ ID NO: 21864 - protein, 9 aa, synthetic construct
GGSGEDFVF

SEQ ID NO: 21865 - protein, 9 aa, synthetic construct
GGAGNDNLH

SEQ ID NO: 21866 - protein, 9 aa, synthetic construct
GGSGEDDMS

SEQ ID NO: 21867 - protein, 9 aa, synthetic construct
GGSGEDDLS

SEQ ID NO: 21868 - protein, 9 aa, synthetic construct
GGSGEDDLK

SEQ ID NO: 21869 - protein, 9 aa, synthetic construct
GGAGNDNMA

SEQ ID NO: 21870 - protein, 9 aa, synthetic construct
GGSGEDALT

SEQ ID NO: 21871 - protein, 9 aa, synthetic construct
GGSGDDYVN

SEQ ID NO: 21872 - protein, 9 aa, synthetic construct
GGAGNDNMN

SEQ ID NO: 21873 - protein, 9 aa, synthetic construct
GGSGGDELD

SEQ ID NO: 21874 - protein, 9 aa, synthetic construct
GGSGGDELV

SEQ ID NO: 21875 - protein, 9 aa, synthetic construct
GGSGGDFIF

SEQ ID NO: 21876 - protein, 9 aa, synthetic construct
GGAGNDIMY

SEQ ID NO: 21877 - protein, 9 aa, synthetic construct
GGAGNDIAL

SEQ ID NO: 21878 - protein, 9 aa, synthetic construct
GGSGHDTLA

SEQ ID NO: 21879 - protein, 9 aa, synthetic construct
GGAGNDIAV

SEQ ID NO: 21880 - protein, 9 aa, synthetic construct
GGSGHDTII

SEQ ID NO: 21881 - protein, 9 aa, synthetic construct
GGSGHDSLR

SEQ ID NO: 21882 - protein, 9 aa, synthetic construct
GGSGHDSLQ

SEQ ID NO: 21883 - protein, 9 aa, synthetic construct
GGSGHDSLI

SEQ ID NO: 21884 - protein, 9 aa, synthetic construct
GGSGHDSLG

SEQ ID NO: 21885 - protein, 9 aa, synthetic construct
GGSGHDSFV

SEQ ID NO: 21886 - protein, 9 aa, synthetic construct
GGSGHDRVY

SEQ ID NO: 21887 - protein, 9 aa, synthetic construct
GGSGHDRVK

SEQ ID NO: 21888 - protein, 9 aa, synthetic construct
GGSGHDRVD

SEQ ID NO: 21889 - protein, 9 aa, synthetic construct
GGSGHDRIS

SEQ ID NO: 21890 - protein, 9 aa, synthetic construct
GGSGHDLVQ

SEQ ID NO: 21891 - protein, 9 aa, synthetic construct
GGSGHDLIY

SEQ ID NO: 21892 - protein, 9 aa, synthetic construct
GGSGHDLFV

SEQ ID NO: 21893 - protein, 9 aa, synthetic construct
GGSGHDKIY

SEQ ID NO: 21894 - protein, 9 aa, synthetic construct
GGSGHDIMN

SEQ ID NO: 21895 - protein, 9 aa, synthetic construct
GGSGHDILV

SEQ ID NO: 21896 - protein, 9 aa, synthetic construct
GGSGHDILT

SEQ ID NO: 21897 - protein, 9 aa, synthetic construct
GGSGHDILI

SEQ ID NO: 21898 - protein, 9 aa, synthetic construct
GGAGNDIML

SEQ ID NO: 21899 - protein, 9 aa, synthetic construct
GGSGHDIIT

SEQ ID NO: 21900 - protein, 9 aa, synthetic construct
GGSGHDIID

SEQ ID NO: 21901 - protein, 9 aa, synthetic construct
GGSGHDGLG

SEQ ID NO: 21902 - protein, 9 aa, synthetic construct
GGFGQDTIV

SEQ ID NO: 21903 - protein, 9 aa, synthetic construct
GGSGHDTVD

SEQ ID NO: 21904 - protein, 9 aa, synthetic construct
GGSGHDTVI

SEQ ID NO: 21905 - protein, 9 aa, synthetic construct
GGSGHDYLE

SEQ ID NO: 21906 - protein, 9 aa, synthetic construct
GGAGNDHIF

SEQ ID NO: 21907 - protein, 9 aa, synthetic construct
GGEGKDILQ

SEQ ID NO: 21908 - protein, 9 aa, synthetic construct
GGAGNDHII

SEQ ID NO: 21909 - protein, 9 aa, synthetic construct
GGAGNDHIQ

SEQ ID NO: 21910 - protein, 9 aa, synthetic construct
GGAGNDHIR

SEQ ID NO: 21911 - protein, 9 aa, synthetic construct
GGFGPDTID

SEQ ID NO: 21912 - protein, 9 aa, synthetic construct
GGSGIDEAF

SEQ ID NO: 21913 - protein, 9 aa, synthetic construct
GGSGIDALF

SEQ ID NO: 21914 - protein, 9 aa, synthetic construct
GGSGIDAIT

SEQ ID NO: 21915 - protein, 9 aa, synthetic construct
GGEGKDILI

SEQ ID NO: 21916 - protein, 9 aa, synthetic construct
GGAGNDHLK

SEQ ID NO: 21917 - protein, 9 aa, synthetic construct
GGFGQDELS

SEQ ID NO: 21918 - protein, 9 aa, synthetic construct
GGSGHDTVQ

SEQ ID NO: 21919 - protein, 9 aa, synthetic construct
GGSGHDWLT

SEQ ID NO: 21920 - protein, 9 aa, synthetic construct
GGSGHDWLL

SEQ ID NO: 21921 - protein, 9 aa, synthetic construct
GGSGHDWLD

SEQ ID NO: 21922 - protein, 9 aa, synthetic construct
GGSGHDVVI

SEQ ID NO: 21923 - protein, 9 aa, synthetic construct
GGSGHDVMK

SEQ ID NO: 21924 - protein, 9 aa, synthetic construct
GGSGHDVLY

SEQ ID NO: 21925 - protein, 9 aa, synthetic construct
GGEGKDILE

SEQ ID NO: 21926 - protein, 9 aa, synthetic construct
GGSGHDVLL

SEQ ID NO: 21927 - protein, 9 aa, synthetic construct
GGSGHDVLI

SEQ ID NO: 21928 - protein, 9 aa, synthetic construct
GGFGQDILI

SEQ ID NO: 21929 - protein, 9 aa, synthetic construct
GGFGQDLIN

SEQ ID NO: 21930 - protein, 9 aa, synthetic construct
GGSGHDELY

SEQ ID NO: 21931 - protein, 9 aa, synthetic construct
GGSGHDELR

SEQ ID NO: 21932 - protein, 9 aa, synthetic construct
GGSGGDFLD

SEQ ID NO: 21933 - protein, 9 aa, synthetic construct
GGAGNDIVL

SEQ ID NO: 21934 - protein, 9 aa, synthetic construct
GGSGGDRFF

SEQ ID NO: 21935 - protein, 9 aa, synthetic construct
GGSGGDQLS

SEQ ID NO: 21936 - protein, 9 aa, synthetic construct
GGSGGDQIY

SEQ ID NO: 21937 - protein, 9 aa, synthetic construct
GGEGKDALN

SEQ ID NO: 21938 - protein, 9 aa, synthetic construct
GGEGIDYLF

SEQ ID NO: 21939 - protein, 9 aa, synthetic construct
GGSGGDMLS

SEQ ID NO: 21940 - protein, 9 aa, synthetic construct
GGEGIDYIG

SEQ ID NO: 21941 - protein, 9 aa, synthetic construct
GGFGRDLLK

SEQ ID NO: 21942 - protein, 9 aa, synthetic construct
GGSGGDLLV

SEQ ID NO: 21943 - protein, 9 aa, synthetic construct
GGSGGDLLS

SEQ ID NO: 21944 - protein, 9 aa, synthetic construct
GGAGNDKVF

SEQ ID NO: 21945 - protein, 9 aa, synthetic construct
GGSGGDLLA

SEQ ID NO: 21946 - protein, 9 aa, synthetic construct
GGAGNDKYR

SEQ ID NO: 21947 - protein, 9 aa, synthetic construct
GGSGGDLID

SEQ ID NO: 21948 - protein, 9 aa, synthetic construct
GGSGGDKYL

SEQ ID NO: 21949 - protein, 9 aa, synthetic construct
GGAGNDLAL

SEQ ID NO: 21950 - protein, 9 aa, synthetic construct
GGAGNDLAS

SEQ ID NO: 21951 - protein, 9 aa, synthetic construct
GGAGNDLAV

SEQ ID NO: 21952 - protein, 9 aa, synthetic construct
GGEGIDVVN

SEQ ID NO: 21953 - protein, 9 aa, synthetic construct
GGAGNDLFE

SEQ ID NO: 21954 - protein, 9 aa, synthetic construct
GGSGGDILD

SEQ ID NO: 21955 - protein, 9 aa, synthetic construct
GGSGGDIFV

SEQ ID NO: 21956 - protein, 9 aa, synthetic construct
GGSGGDIAL

SEQ ID NO: 21957 - protein, 9 aa, synthetic construct
GGSGGDHVV

SEQ ID NO: 21958 - protein, 9 aa, synthetic construct
GGSGGDGIW

SEQ ID NO: 21959 - protein, 9 aa, synthetic construct
GGSGGDRLF

SEQ ID NO: 21960 - protein, 9 aa, synthetic construct
GGAGNDKLQ

SEQ ID NO: 21961 - protein, 9 aa, synthetic construct
GGSGGDRLY

SEQ ID NO: 21962 - protein, 9 aa, synthetic construct
GGSGGDVIY

SEQ ID NO: 21963 - protein, 9 aa, synthetic construct
GGAGNDIVQ

SEQ ID NO: 21964 - protein, 9 aa, synthetic construct
GGAGNDIVV

SEQ ID NO: 21965 - protein, 9 aa, synthetic construct
GGSGHDALH

SEQ ID NO: 21966 - protein, 9 aa, synthetic construct
GGSGGDYLH

SEQ ID NO: 21967 - protein, 9 aa, synthetic construct
GGAGNDIYN

SEQ ID NO: 21968 - protein, 9 aa, synthetic construct
GGAGNDIYS

SEQ ID NO: 21969 - protein, 9 aa, synthetic construct
GGFGQDYLD

SEQ ID NO: 21970 - protein, 9 aa, synthetic construct
GGAGNDKFI

SEQ ID NO: 21971 - protein, 9 aa, synthetic construct
GGSGGDVLR

SEQ ID NO: 21972 - protein, 9 aa, synthetic construct
GGSGGDVLD

SEQ ID NO: 21973 - protein, 9 aa, synthetic construct
GGAGNDKFV

SEQ ID NO: 21974 - protein, 9 aa, synthetic construct
GGSGGDVFV

SEQ ID NO: 21975 - protein, 9 aa, synthetic construct
GGAGNDKLK

SEQ ID NO: 21976 - protein, 9 aa, synthetic construct
GGAGNDKIH

SEQ ID NO: 21977 - protein, 9 aa, synthetic construct
GGSGGDTMR

SEQ ID NO: 21978 - protein, 9 aa, synthetic construct
GGFGRDIFR

SEQ ID NO: 21979 - protein, 9 aa, synthetic construct
GGSGGDTLK

SEQ ID NO: 21980 - protein, 9 aa, synthetic construct
GGEGKDALT

SEQ ID NO: 21981 - protein, 9 aa, synthetic construct
GGSGGDTII

SEQ ID NO: 21982 - protein, 9 aa, synthetic construct
GGSGGDTAR

SEQ ID NO: 21983 - protein, 9 aa, synthetic construct
GGSGGDSLV

SEQ ID NO: 21984 - protein, 9 aa, synthetic construct
GGSGGDSLS

SEQ ID NO: 21985 - protein, 9 aa, synthetic construct
GGSGGDSLI

SEQ ID NO: 21986 - protein, 9 aa, synthetic construct
GGAGNDKLG

SEQ ID NO: 21987 - protein, 9 aa, synthetic construct
GGSGDDVVS

SEQ ID NO: 21988 - protein, 9 aa, synthetic construct
GGSGDDVVQ

SEQ ID NO: 21989 - protein, 9 aa, synthetic construct
GGAGNDQII

SEQ ID NO: 21990 - protein, 9 aa, synthetic construct
GGSGADVVL

SEQ ID NO: 21991 - protein, 9 aa, synthetic construct
GGSGDDDLN

SEQ ID NO: 21992 - protein, 9 aa, synthetic construct
GGSGDDDIY

SEQ ID NO: 21993 - protein, 9 aa, synthetic construct
GGSGDDDIG

SEQ ID NO: 21994 - protein, 9 aa, synthetic construct
GGSGDDCIR

SEQ ID NO: 21995 - protein, 9 aa, synthetic construct
GGSGDDAYV

SEQ ID NO: 21996 - protein, 9 aa, synthetic construct
GGSGDDAVH

SEQ ID NO: 21997 - protein, 9 aa, synthetic construct
GGAGNDSVV

SEQ ID NO: 21998 - protein, 9 aa, synthetic construct
GGSGDDAMF

SEQ ID NO: 21999 - protein, 9 aa, synthetic construct
GGSGDDALT

SEQ ID NO: 22000 - protein, 9 aa, synthetic construct
GGSGDDALQ

SEQ ID NO: 22001 - protein, 9 aa, synthetic construct
GGEGIDLLY

SEQ ID NO: 22002 - protein, 9 aa, synthetic construct
GGFGSDVID

SEQ ID NO: 22003 - protein, 9 aa, synthetic construct
GGSGDDALA

SEQ ID NO: 22004 - protein, 9 aa, synthetic construct
GGSGDDAIF

SEQ ID NO: 22005 - protein, 9 aa, synthetic construct
GGSGDDAAD

SEQ ID NO: 22006 - protein, 9 aa, synthetic construct
GGSGADYMS

SEQ ID NO: 22007 - protein, 9 aa, synthetic construct
GGAGNDTAN

SEQ ID NO: 22008 - protein, 9 aa, synthetic construct
GGAGNDTAT

SEQ ID NO: 22009 - protein, 9 aa, synthetic construct
GGSGADYIG

SEQ ID NO: 22010 - protein, 9 aa, synthetic construct
GGSGADWLT

SEQ ID NO: 22011 - protein, 9 aa, synthetic construct
GGSGADWLE

SEQ ID NO: 22012 - protein, 9 aa, synthetic construct
GGSGADWIS

SEQ ID NO: 22013 - protein, 9 aa, synthetic construct
GGSGADVYI

SEQ ID NO: 22014 - protein, 9 aa, synthetic construct
GGAGNDTFM

SEQ ID NO: 22015 - protein, 9 aa, synthetic construct
GGSGADVVY

SEQ ID NO: 22016 - protein, 9 aa, synthetic construct
GGSGDDDLW

SEQ ID NO: 22017 - protein, 9 aa, synthetic construct
GGAGNDSMQ

SEQ ID NO: 22018 - protein, 9 aa, synthetic construct
GGSGDDDVF

SEQ ID NO: 22019 - protein, 9 aa, synthetic construct
GGSGDDFLV

SEQ ID NO: 22020 - protein, 9 aa, synthetic construct
GGSGDDHLT

SEQ ID NO: 22021 - protein, 9 aa, synthetic construct
GGSGDDHLA

SEQ ID NO: 22022 - protein, 9 aa, synthetic construct
GGSGDDHIS

SEQ ID NO: 22023 - protein, 9 aa, synthetic construct
GGSGDDHIE

SEQ ID NO: 22024 - protein, 9 aa, synthetic construct
GGSGDDHID

SEQ ID NO: 22025 - protein, 9 aa, synthetic construct
GGSGDDGLR

SEQ ID NO: 22026 - protein, 9 aa, synthetic construct
GGAGNDSIH

SEQ ID NO: 22027 - protein, 9 aa, synthetic construct
GGSGDDFVS

SEQ ID NO: 22028 - protein, 9 aa, synthetic construct
GGSGDDFVH

SEQ ID NO: 22029 - protein, 9 aa, synthetic construct
GGSGDDFVF

SEQ ID NO: 22030 - protein, 9 aa, synthetic construct
GGAGNDSLC

SEQ ID NO: 22031 - protein, 9 aa, synthetic construct
GGSGDDFLK

SEQ ID NO: 22032 - protein, 9 aa, synthetic construct
GGFGSDTLY

SEQ ID NO: 22033 - protein, 9 aa, synthetic construct
GGSGDDFLF

SEQ ID NO: 22034 - protein, 9 aa, synthetic construct
GGSGDDFIY

SEQ ID NO: 22035 - protein, 9 aa, synthetic construct
GGSGDDFIL

SEQ ID NO: 22036 - protein, 9 aa, synthetic construct
GGSGDDFIK

SEQ ID NO: 22037 - protein, 9 aa, synthetic construct
GGSGDDELI

SEQ ID NO: 22038 - protein, 9 aa, synthetic construct
GGSGDDEIF

SEQ ID NO: 22039 - protein, 9 aa, synthetic construct
GGSGDDEIE

SEQ ID NO: 22040 - protein, 9 aa, synthetic construct
GGSGDDEFV

SEQ ID NO: 22041 - protein, 9 aa, synthetic construct
GGSGDDDYV

SEQ ID NO: 22042 - protein, 9 aa, synthetic construct
GGSGDDDVY

SEQ ID NO: 22043 - protein, 9 aa, synthetic construct
GGSGDDDVT

SEQ ID NO: 22044 - protein, 9 aa, synthetic construct
GGSGADVVT

SEQ ID NO: 22045 - protein, 9 aa, synthetic construct
GGSGADVMT

SEQ ID NO: 22046 - protein, 9 aa, synthetic construct
GGAGNDSFL

SEQ ID NO: 22047 - protein, 9 aa, synthetic construct
GGSGADVMR

SEQ ID NO: 22048 - protein, 9 aa, synthetic construct
GGSGADRYR

SEQ ID NO: 22049 - protein, 9 aa, synthetic construct
GGSGADRMY

SEQ ID NO: 22050 - protein, 9 aa, synthetic construct
GGFGSDWVL

SEQ ID NO: 22051 - protein, 9 aa, synthetic construct
GGSGADRML

SEQ ID NO: 22052 - protein, 9 aa, synthetic construct
GGSGADRLW

SEQ ID NO: 22053 - protein, 9 aa, synthetic construct
GGSGADRII

SEQ ID NO: 22054 - protein, 9 aa, synthetic construct
GGSGADRFR

SEQ ID NO: 22055 - protein, 9 aa, synthetic construct
GGSGADRFM

SEQ ID NO: 22056 - protein, 9 aa, synthetic construct
GGSGADRFL

SEQ ID NO: 22057 - protein, 9 aa, synthetic construct
GGSGADRAS

SEQ ID NO: 22058 - protein, 9 aa, synthetic construct
GGSGADQVS

SEQ ID NO: 22059 - protein, 9 aa, synthetic construct
GGAGNDTYD

SEQ ID NO: 22060 - protein, 9 aa, synthetic construct
GGSGADQLW

SEQ ID NO: 22061 - protein, 9 aa, synthetic construct
GGSGADQLN

SEQ ID NO: 22062 - protein, 9 aa, synthetic construct
GGSGADQIF

SEQ ID NO: 22063 - protein, 9 aa, synthetic construct
GGSGADQFR

SEQ ID NO: 22064 - protein, 9 aa, synthetic construct
GGSGADQFQ

SEQ ID NO: 22065 - protein, 9 aa, synthetic construct
GGSGADQFN

SEQ ID NO: 22066 - protein, 9 aa, synthetic construct
GGSGADNLS

SEQ ID NO: 22067 - protein, 9 aa, synthetic construct
GGSGADNLR

SEQ ID NO: 22068 - protein, 9 aa, synthetic construct
GGEGIDKIF

SEQ ID NO: 22069 - protein, 9 aa, synthetic construct
GGAGNDVAI

SEQ ID NO: 22070 - protein, 9 aa, synthetic construct
GGSGADMMD

SEQ ID NO: 22071 - protein, 9 aa, synthetic construct
GGSGADMLT

SEQ ID NO: 22072 - protein, 9 aa, synthetic construct
GGSGADMLA

SEQ ID NO: 22073 - protein, 9 aa, synthetic construct
GGSGADRYT

SEQ ID NO: 22074 - protein, 9 aa, synthetic construct
GGSGADSIA

SEQ ID NO: 22075 - protein, 9 aa, synthetic construct
GGSGADSIE

SEQ ID NO: 22076 - protein, 9 aa, synthetic construct
GGSGADTVT

SEQ ID NO: 22077 - protein, 9 aa, synthetic construct
GGSGADVML

SEQ ID NO: 22078 - protein, 9 aa, synthetic construct
GGSGADVMA

SEQ ID NO: 22079 - protein, 9 aa, synthetic construct
GGSGADVLY

SEQ ID NO: 22080 - protein, 9 aa, synthetic construct
GGAGNDTFW

SEQ ID NO: 22081 - protein, 9 aa, synthetic construct
GGSGADVLG

SEQ ID NO: 22082 - protein, 9 aa, synthetic construct
GGSGADVIS

SEQ ID NO: 22083 - protein, 9 aa, synthetic construct
GGSGADVIA

SEQ ID NO: 22084 - protein, 9 aa, synthetic construct
GGSGADVFT

SEQ ID NO: 22085 - protein, 9 aa, synthetic construct
GGSGADVFI

SEQ ID NO: 22086 - protein, 9 aa, synthetic construct
GGSGADVFH

SEQ ID NO: 22087 - protein, 9 aa, synthetic construct
GGSGADTYT

SEQ ID NO: 22088 - protein, 9 aa, synthetic construct
GGSGADTVR

SEQ ID NO: 22089 - protein, 9 aa, synthetic construct
GGSGADSIQ

SEQ ID NO: 22090 - protein, 9 aa, synthetic construct
GGSGADTVF

SEQ ID NO: 22091 - protein, 9 aa, synthetic construct
GGSGADTVA

SEQ ID NO: 22092 - protein, 9 aa, synthetic construct
GGSGADTMK

SEQ ID NO: 22093 - protein, 9 aa, synthetic construct
GGSGADTLG

SEQ ID NO: 22094 - protein, 9 aa, synthetic construct
GGSGADTIR

SEQ ID NO: 22095 - protein, 9 aa, synthetic construct
GGSGADTIQ

SEQ ID NO: 22096 - protein, 9 aa, synthetic construct
GGSGADTFH

SEQ ID NO: 22097 - protein, 9 aa, synthetic construct
GGSGADTFE

SEQ ID NO: 22098 - protein, 9 aa, synthetic construct
GGSGADSVL

SEQ ID NO: 22099 - protein, 9 aa, synthetic construct
GGSGADSVD

SEQ ID NO: 22100 - protein, 9 aa, synthetic construct
GGSGADSLQ

SEQ ID NO: 22101 - protein, 9 aa, synthetic construct
GGSGDDHLV

SEQ ID NO: 22102 - protein, 9 aa, synthetic construct
GGSGDDIFF

SEQ ID NO: 22103 - protein, 9 aa, synthetic construct
GGAGNDQIK

SEQ ID NO: 22104 - protein, 9 aa, synthetic construct
GGSGDDRFD

SEQ ID NO: 22105 - protein, 9 aa, synthetic construct
GGSGDDSLQ

SEQ ID NO: 22106 - protein, 9 aa, synthetic construct
GGSGDDSLM

SEQ ID NO: 22107 - protein, 9 aa, synthetic construct
GGAGNDQVK

SEQ ID NO: 22108 - protein, 9 aa, synthetic construct
GGSGDDSLE

SEQ ID NO: 22109 - protein, 9 aa, synthetic construct
GGSGDDSLC

SEQ ID NO: 22110 - protein, 9 aa, synthetic construct
GGSGDDSIY

SEQ ID NO: 22111 - protein, 9 aa, synthetic construct
GGSGDDSIW

SEQ ID NO: 22112 - protein, 9 aa, synthetic construct
GGSGDDSIS

SEQ ID NO: 22113 - protein, 9 aa, synthetic construct
GGFGSDLVN

SEQ ID NO: 22114 - protein, 9 aa, synthetic construct
GGSGDDSIG

SEQ ID NO: 22115 - protein, 9 aa, synthetic construct
GGSGDDSIE

SEQ ID NO: 22116 - protein, 9 aa, synthetic construct
GGFGSDNMS

SEQ ID NO: 22117 - protein, 9 aa, synthetic construct
GGAGNDQYH

SEQ ID NO: 22118 - protein, 9 aa, synthetic construct
GGAGNDQYL

SEQ ID NO: 22119 - protein, 9 aa, synthetic construct
GGFGSDQLQ

SEQ ID NO: 22120 - protein, 9 aa, synthetic construct
GGSGDDSAE

SEQ ID NO: 22121 - protein, 9 aa, synthetic construct
GGAGNDQYW

SEQ ID NO: 22122 - protein, 9 aa, synthetic construct
GGEGIDRLS

SEQ ID NO: 22123 - protein, 9 aa, synthetic construct
GGSGDDRYI

SEQ ID NO: 22124 - protein, 9 aa, synthetic construct
GGAGNDRAI

SEQ ID NO: 22125 - protein, 9 aa, synthetic construct
GGAGNDRAR

SEQ ID NO: 22126 - protein, 9 aa, synthetic construct
GGEGIDRLI

SEQ ID NO: 22127 - protein, 9 aa, synthetic construct
GGSGDDRLW

SEQ ID NO: 22128 - protein, 9 aa, synthetic construct
GGSGDDRIT

SEQ ID NO: 22129 - protein, 9 aa, synthetic construct
GGSGDDRIL

SEQ ID NO: 22130 - protein, 9 aa, synthetic construct
GGAGNDQVI

SEQ ID NO: 22131 - protein, 9 aa, synthetic construct
GGSGDDSMH

SEQ ID NO: 22132 - protein, 9 aa, synthetic construct
GGSGDDSVF

SEQ ID NO: 22133 - protein, 9 aa, synthetic construct
GGSGDDTML

SEQ ID NO: 22134 - protein, 9 aa, synthetic construct
GGSGDDVVF

SEQ ID NO: 22135 - protein, 9 aa, synthetic construct
GGSGDDVLW

SEQ ID NO: 22136 - protein, 9 aa, synthetic construct
GGSGDDVLC

SEQ ID NO: 22137 - protein, 9 aa, synthetic construct
GGSGDDVFD

SEQ ID NO: 22138 - protein, 9 aa, synthetic construct
GGSGDDVAV

SEQ ID NO: 22139 - protein, 9 aa, synthetic construct
GGSGDDTYH

SEQ ID NO: 22140 - protein, 9 aa, synthetic construct
GGSGDDTVG

SEQ ID NO: 22141 - protein, 9 aa, synthetic construct
GGSGDDTVF

SEQ ID NO: 22142 - protein, 9 aa, synthetic construct
GGSGDDTVE

SEQ ID NO: 22143 - protein, 9 aa, synthetic construct
GGSGDDTMV

SEQ ID NO: 22144 - protein, 9 aa, synthetic construct
GGSGDDTMR

SEQ ID NO: 22145 - protein, 9 aa, synthetic construct
GGAGNDQMA

SEQ ID NO: 22146 - protein, 9 aa, synthetic construct
GGSGDDSVN

SEQ ID NO: 22147 - protein, 9 aa, synthetic construct
GGSGDDTMG

SEQ ID NO: 22148 - protein, 9 aa, synthetic construct
GGSGDDTLG

SEQ ID NO: 22149 - protein, 9 aa, synthetic construct
GGSGDDTIW

SEQ ID NO: 22150 - protein, 9 aa, synthetic construct
GGSGDDTIK

SEQ ID NO: 22151 - protein, 9 aa, synthetic construct
GGSGDDTIG

SEQ ID NO: 22152 - protein, 9 aa, synthetic construct
GGAGNDQMI

SEQ ID NO: 22153 - protein, 9 aa, synthetic construct
GGFGSDLLD

SEQ ID NO: 22154 - protein, 9 aa, synthetic construct
GGSGDDTAA

SEQ ID NO: 22155 - protein, 9 aa, synthetic construct
GGSGDDSYY

SEQ ID NO: 22156 - protein, 9 aa, synthetic construct
GGSGDDSYI

SEQ ID NO: 22157 - protein, 9 aa, synthetic construct
GGSGDDSVY

SEQ ID NO: 22158 - protein, 9 aa, synthetic construct
GGEGIDRFA

SEQ ID NO: 22159 - protein, 9 aa, synthetic construct
GGSGDDQLM

SEQ ID NO: 22160 - protein, 9 aa, synthetic construct
GGSGDDIIH

SEQ ID NO: 22161 - protein, 9 aa, synthetic construct
GGSGDDQLH

SEQ ID NO: 22162 - protein, 9 aa, synthetic construct
GGSGDDLAD

SEQ ID NO: 22163 - protein, 9 aa, synthetic construct
GGAGNDRVS

SEQ ID NO: 22164 - protein, 9 aa, synthetic construct
GGSGDDKLV

SEQ ID NO: 22165 - protein, 9 aa, synthetic construct
GGSGDDKIY

SEQ ID NO: 22166 - protein, 9 aa, synthetic construct
GGAGNDRYD

SEQ ID NO: 22167 - protein, 9 aa, synthetic construct
GGSGDDKIT

SEQ ID NO: 22168 - protein, 9 aa, synthetic construct
GGSGDDKIS

SEQ ID NO: 22169 - protein, 9 aa, synthetic construct
GGSGDDKIK

SEQ ID NO: 22170 - protein, 9 aa, synthetic construct
GGAGNDRYL

SEQ ID NO: 22171 - protein, 9 aa, synthetic construct
GGAGNDRYQ

SEQ ID NO: 22172 - protein, 9 aa, synthetic construct
GGSGDDIYY

SEQ ID NO: 22173 - protein, 9 aa, synthetic construct
GGSGDDIYV

SEQ ID NO: 22174 - protein, 9 aa, synthetic construct
GGFGSDTAT

SEQ ID NO: 22175 - protein, 9 aa, synthetic construct
GGFGSDTFL

SEQ ID NO: 22176 - protein, 9 aa, synthetic construct
GGSGDDIYD

SEQ ID NO: 22177 - protein, 9 aa, synthetic construct
GGSGDDIVY

SEQ ID NO: 22178 - protein, 9 aa, synthetic construct
GGFGSDTID

SEQ ID NO: 22179 - protein, 9 aa, synthetic construct
GGFGSDTIE

SEQ ID NO: 22180 - protein, 9 aa, synthetic construct
GGSGDDIVD

SEQ ID NO: 22181 - protein, 9 aa, synthetic construct
GGFGSDTLD

SEQ ID NO: 22182 - protein, 9 aa, synthetic construct
GGSGDDIMN

SEQ ID NO: 22183 - protein, 9 aa, synthetic construct
GGSGDDILH

SEQ ID NO: 22184 - protein, 9 aa, synthetic construct
GGSGDDIIS

SEQ ID NO: 22185 - protein, 9 aa, synthetic construct
GGSGDDIIQ

SEQ ID NO: 22186 - protein, 9 aa, synthetic construct
GGSGDDIII

SEQ ID NO: 22187 - protein, 9 aa, synthetic construct
GGAGNDRVI

SEQ ID NO: 22188 - protein, 9 aa, synthetic construct
GGSGDDLFI

SEQ ID NO: 22189 - protein, 9 aa, synthetic construct
GGSGDDLIG

SEQ ID NO: 22190 - protein, 9 aa, synthetic construct
GGSGDDLYY

SEQ ID NO: 22191 - protein, 9 aa, synthetic construct
GGAGNDRIK

SEQ ID NO: 22192 - protein, 9 aa, synthetic construct
GGSGDDQIW

SEQ ID NO: 22193 - protein, 9 aa, synthetic construct
GGSGDDQIN

SEQ ID NO: 22194 - protein, 9 aa, synthetic construct
GGSGDDQID

SEQ ID NO: 22195 - protein, 9 aa, synthetic construct
GGAGNDRLC

SEQ ID NO: 22196 - protein, 9 aa, synthetic construct
GGSGDDNLT

SEQ ID NO: 22197 - protein, 9 aa, synthetic construct
GGSGDDNLL

SEQ ID NO: 22198 - protein, 9 aa, synthetic construct
GGSGDDNIS

SEQ ID NO: 22199 - protein, 9 aa, synthetic construct
GGSGDDNID

SEQ ID NO: 22200 - protein, 9 aa, synthetic construct
GGFGSDSIT

SEQ ID NO: 22201 - protein, 9 aa, synthetic construct
GGSGDDMAR

SEQ ID NO: 22202 - protein, 9 aa, synthetic construct
GGSGDDLYL

SEQ ID NO: 22203 - protein, 9 aa, synthetic construct
GGSGDDLII

SEQ ID NO: 22204 - protein, 9 aa, synthetic construct
GGSGDDLYH

SEQ ID NO: 22205 - protein, 9 aa, synthetic construct
GGSGDDLVS

SEQ ID NO: 22206 - protein, 9 aa, synthetic construct
GGAGNDRMR

SEQ ID NO: 22207 - protein, 9 aa, synthetic construct
GGSGDDLVF

SEQ ID NO: 22208 - protein, 9 aa, synthetic construct
GGSGDDLVE

SEQ ID NO: 22209 - protein, 9 aa, synthetic construct
GGSGDDLML

SEQ ID NO: 22210 - protein, 9 aa, synthetic construct
GGSGDDLMF

SEQ ID NO: 22211 - protein, 9 aa, synthetic construct
GGAGNDRVA

SEQ ID NO: 22212 - protein, 9 aa, synthetic construct
GGSGDDLLM

SEQ ID NO: 22213 - protein, 9 aa, synthetic construct
GGSGDDLIQ

SEQ ID NO: 22214 - protein, 9 aa, synthetic construct
GGSGDDLIN

SEQ ID NO: 22215 - protein, 9 aa, synthetic construct
GGSGIDILN

SEQ ID NO: 22216 - protein, 9 aa, synthetic construct
GGSGIDKIV

SEQ ID NO: 22217 - protein, 9 aa, synthetic construct
GGSGIDKLF

SEQ ID NO: 22218 - protein, 9 aa, synthetic construct
GGSGNDRFF

SEQ ID NO: 22219 - protein, 9 aa, synthetic construct
GGSGNDSIK

SEQ ID NO: 22220 - protein, 9 aa, synthetic construct
GGAGLDTYV

SEQ ID NO: 22221 - protein, 9 aa, synthetic construct
GGFGNDLLV

SEQ ID NO: 22222 - protein, 9 aa, synthetic construct
GGSGNDSFM

SEQ ID NO: 22223 - protein, 9 aa, synthetic construct
GGAGLDVAS

SEQ ID NO: 22224 - protein, 9 aa, synthetic construct
GGSGNDSAF

SEQ ID NO: 22225 - protein, 9 aa, synthetic construct
GGSGNDRYI

SEQ ID NO: 22226 - protein, 9 aa, synthetic construct
GGEGKDTVS

SEQ ID NO: 22227 - protein, 9 aa, synthetic construct
GGSGNDRVS

SEQ ID NO: 22228 - protein, 9 aa, synthetic construct
GGAGLDVFL

SEQ ID NO: 22229 - protein, 9 aa, synthetic construct
GGSGNDRVN

SEQ ID NO: 22230 - protein, 9 aa, synthetic construct
GGSGNDRVD

SEQ ID NO: 22231 - protein, 9 aa, synthetic construct
GGSGNDRMT

SEQ ID NO: 22232 - protein, 9 aa, synthetic construct
GGSGNDRMS

SEQ ID NO: 22233 - protein, 9 aa, synthetic construct
GGFGNDLVN

SEQ ID NO: 22234 - protein, 9 aa, synthetic construct
GGSGNDRMQ

SEQ ID NO: 22235 - protein, 9 aa, synthetic construct
GGFGNDLVQ

SEQ ID NO: 22236 - protein, 9 aa, synthetic construct
GGEGKDTVN

SEQ ID NO: 22237 - protein, 9 aa, synthetic construct
GGFGNDLVY

SEQ ID NO: 22238 - protein, 9 aa, synthetic construct
GGSGNDRLM

SEQ ID NO: 22239 - protein, 9 aa, synthetic construct
GGSGNDRLG

SEQ ID NO: 22240 - protein, 9 aa, synthetic construct
GGEGKDTLY

SEQ ID NO: 22241 - protein, 9 aa, synthetic construct
GGAGLDVLI

SEQ ID NO: 22242 - protein, 9 aa, synthetic construct
GGAGLDVLN

SEQ ID NO: 22243 - protein, 9 aa, synthetic construct
GGAGLDVLQ

SEQ ID NO: 22244 - protein, 9 aa, synthetic construct
GGSGNDSIQ

SEQ ID NO: 22245 - protein, 9 aa, synthetic construct
GGSGNDSIV

SEQ ID NO: 22246 - protein, 9 aa, synthetic construct
GGSGNDSME

SEQ ID NO: 22247 - protein, 9 aa, synthetic construct
GGSGNDTAW

SEQ ID NO: 22248 - protein, 9 aa, synthetic construct
GGSGNDTYK

SEQ ID NO: 22249 - protein, 9 aa, synthetic construct
GGSGNDTVW

SEQ ID NO: 22250 - protein, 9 aa, synthetic construct
GGSGNDTVR

SEQ ID NO: 22251 - protein, 9 aa, synthetic construct
GGFGNDLIN

SEQ ID NO: 22252 - protein, 9 aa, synthetic construct
GGSGNDTVF

SEQ ID NO: 22253 - protein, 9 aa, synthetic construct
GGSGNDTVC

SEQ ID NO: 22254 - protein, 9 aa, synthetic construct
GGSGNDTMW

SEQ ID NO: 22255 - protein, 9 aa, synthetic construct
GGSGNDTMQ

SEQ ID NO: 22256 - protein, 9 aa, synthetic construct
GGSGNDTMH

SEQ ID NO: 22257 - protein, 9 aa, synthetic construct
GGSGNDTIK

SEQ ID NO: 22258 - protein, 9 aa, synthetic construct
GGSGNDTFA

SEQ ID NO: 22259 - protein, 9 aa, synthetic construct
GGSGNDTAV

SEQ ID NO: 22260 - protein, 9 aa, synthetic construct
GGSGNDSMT

SEQ ID NO: 22261 - protein, 9 aa, synthetic construct
GGSGNDTAR

SEQ ID NO: 22262 - protein, 9 aa, synthetic construct
GGAGLDTMH

SEQ ID NO: 22263 - protein, 9 aa, synthetic construct
GGSGNDTAL

SEQ ID NO: 22264 - protein, 9 aa, synthetic construct
GGSGNDTAI

SEQ ID NO: 22265 - protein, 9 aa, synthetic construct
GGEGKDVFL

SEQ ID NO: 22266 - protein, 9 aa, synthetic construct
GGSGNDSYR

SEQ ID NO: 22267 - protein, 9 aa, synthetic construct
GGSGNDSYI

SEQ ID NO: 22268 - protein, 9 aa, synthetic construct
GGSGNDSVW

SEQ ID NO: 22269 - protein, 9 aa, synthetic construct
GGSGNDSVN

SEQ ID NO: 22270 - protein, 9 aa, synthetic construct
GGEGKDVAI

SEQ ID NO: 22271 - protein, 9 aa, synthetic construct
GGSGNDSMY

SEQ ID NO: 22272 - protein, 9 aa, synthetic construct
GGAGLDVLS

SEQ ID NO: 22273 - protein, 9 aa, synthetic construct
GGSGNDRFE

SEQ ID NO: 22274 - protein, 9 aa, synthetic construct
GGSGNDVAY

SEQ ID NO: 22275 - protein, 9 aa, synthetic construct
GGAGLDVLY

SEQ ID NO: 22276 - protein, 9 aa, synthetic construct
GGEGKDTIS

SEQ ID NO: 22277 - protein, 9 aa, synthetic construct
GGSGNDMLW

SEQ ID NO: 22278 - protein, 9 aa, synthetic construct
GGSGNDMIN

SEQ ID NO: 22279 - protein, 9 aa, synthetic construct
GGSGNDMID

SEQ ID NO: 22280 - protein, 9 aa, synthetic construct
GGAGMDLID

SEQ ID NO: 22281 - protein, 9 aa, synthetic construct
GGSGNDLVS

SEQ ID NO: 22282 - protein, 9 aa, synthetic construct
GGSGNDLVQ

SEQ ID NO: 22283 - protein, 9 aa, synthetic construct
GGSGNDLVG

SEQ ID NO: 22284 - protein, 9 aa, synthetic construct
GGSGNDLVF

SEQ ID NO: 22285 - protein, 9 aa, synthetic construct
GGSGNDLVE

SEQ ID NO: 22286 - protein, 9 aa, synthetic construct
GGSGNDLMS

SEQ ID NO: 22287 - protein, 9 aa, synthetic construct
GGSGNDLMR

SEQ ID NO: 22288 - protein, 9 aa, synthetic construct
GGEGKDTFS

SEQ ID NO: 22289 - protein, 9 aa, synthetic construct
GGAGMDRLD

SEQ ID NO: 22290 - protein, 9 aa, synthetic construct
GGSGNDLMK

SEQ ID NO: 22291 - protein, 9 aa, synthetic construct
GGSGNDLMD

SEQ ID NO: 22292 - protein, 9 aa, synthetic construct
GGSGNDLMA

SEQ ID NO: 22293 - protein, 9 aa, synthetic construct
GGSGNDLLW

SEQ ID NO: 22294 - protein, 9 aa, synthetic construct
GGAGMDRLK

SEQ ID NO: 22295 - protein, 9 aa, synthetic construct
GGSGNDLAD

SEQ ID NO: 22296 - protein, 9 aa, synthetic construct
GGSGNDKYV

SEQ ID NO: 22297 - protein, 9 aa, synthetic construct
GGSGNDKVN

SEQ ID NO: 22298 - protein, 9 aa, synthetic construct
GGAGMDRLT

SEQ ID NO: 22299 - protein, 9 aa, synthetic construct
GGSGNDKLI

SEQ ID NO: 22300 - protein, 9 aa, synthetic construct
GGSGNDKIW

SEQ ID NO: 22301 - protein, 9 aa, synthetic construct
GGSGNDMVL

SEQ ID NO: 22302 - protein, 9 aa, synthetic construct
GGFGNDRIV

SEQ ID NO: 22303 - protein, 9 aa, synthetic construct
GGFGNDRIS

SEQ ID NO: 22304 - protein, 9 aa, synthetic construct
GGFGNDNLY

SEQ ID NO: 22305 - protein, 9 aa, synthetic construct
GGSGNDQYW

SEQ ID NO: 22306 - protein, 9 aa, synthetic construct
GGSGNDQVS

SEQ ID NO: 22307 - protein, 9 aa, synthetic construct
GGSGNDQVA

SEQ ID NO: 22308 - protein, 9 aa, synthetic construct
GGSGNDQMQ

SEQ ID NO: 22309 - protein, 9 aa, synthetic construct
GGAGLDWIY

SEQ ID NO: 22310 - protein, 9 aa, synthetic construct
GGFGNDNLS

SEQ ID NO: 22311 - protein, 9 aa, synthetic construct
GGSGNDQMD

SEQ ID NO: 22312 - protein, 9 aa, synthetic construct
GGSGNDQMA

SEQ ID NO: 22313 - protein, 9 aa, synthetic construct
GGSGNDQLV

SEQ ID NO: 22314 - protein, 9 aa, synthetic construct
GGSGNDQLQ

SEQ ID NO: 22315 - protein, 9 aa, synthetic construct
GGSGNDQIW

SEQ ID NO: 22316 - protein, 9 aa, synthetic construct
GGFGNDNMQ

SEQ ID NO: 22317 - protein, 9 aa, synthetic construct
GGSGNDNFD

SEQ ID NO: 22318 - protein, 9 aa, synthetic construct
GGFGNDPIA

SEQ ID NO: 22319 - protein, 9 aa, synthetic construct
GGAGLDYLV

SEQ ID NO: 22320 - protein, 9 aa, synthetic construct
GGAGMDALF

SEQ ID NO: 22321 - protein, 9 aa, synthetic construct
GGSGNDNMW

SEQ ID NO: 22322 - protein, 9 aa, synthetic construct
GGEGKDTLI

SEQ ID NO: 22323 - protein, 9 aa, synthetic construct
GGSGNDNLR

SEQ ID NO: 22324 - protein, 9 aa, synthetic construct
GGSGNDNLA

SEQ ID NO: 22325 - protein, 9 aa, synthetic construct
GGSGNDNIS

SEQ ID NO: 22326 - protein, 9 aa, synthetic construct
GGEGKDTLD

SEQ ID NO: 22327 - protein, 9 aa, synthetic construct
GGAGMDGLW

SEQ ID NO: 22328 - protein, 9 aa, synthetic construct
GGAGMDIAD

SEQ ID NO: 22329 - protein, 9 aa, synthetic construct
GGAGLDTLL

SEQ ID NO: 22330 - protein, 9 aa, synthetic construct
GGSGNDVFE

SEQ ID NO: 22331 - protein, 9 aa, synthetic construct
GGAGMDSIM

SEQ ID NO: 22332 - protein, 9 aa, synthetic construct
GGSGQDALD

SEQ ID NO: 22333 - protein, 9 aa, synthetic construct
GGSGQDSLA

SEQ ID NO: 22334 - protein, 9 aa, synthetic construct
GGAGLDILI

SEQ ID NO: 22335 - protein, 9 aa, synthetic construct
GGSGQDSIL

SEQ ID NO: 22336 - protein, 9 aa, synthetic construct
GGAGLDILL

SEQ ID NO: 22337 - protein, 9 aa, synthetic construct
GGAGLDILV

SEQ ID NO: 22338 - protein, 9 aa, synthetic construct
GGFGNDEIK

SEQ ID NO: 22339 - protein, 9 aa, synthetic construct
GGSGQDQLF

SEQ ID NO: 22340 - protein, 9 aa, synthetic construct
GGSGQDQFV

SEQ ID NO: 22341 - protein, 9 aa, synthetic construct
GGEGLDNVY

SEQ ID NO: 22342 - protein, 9 aa, synthetic construct
GGEGLDNLL

SEQ ID NO: 22343 - protein, 9 aa, synthetic construct
GGFGNDELW

SEQ ID NO: 22344 - protein, 9 aa, synthetic construct
GGAGLDLLD

SEQ ID NO: 22345 - protein, 9 aa, synthetic construct
GGSGQDLIW

SEQ ID NO: 22346 - protein, 9 aa, synthetic construct
GGSGQDKIH

SEQ ID NO: 22347 - protein, 9 aa, synthetic construct
GGAGLDLLT

SEQ ID NO: 22348 - protein, 9 aa, synthetic construct
GGSGQDILY

SEQ ID NO: 22349 - protein, 9 aa, synthetic construct
GGSGQDILV

SEQ ID NO: 22350 - protein, 9 aa, synthetic construct
GGSGQDIFY

SEQ ID NO: 22351 - protein, 9 aa, synthetic construct
GGFGNDFIS

SEQ ID NO: 22352 - protein, 9 aa, synthetic construct
GGFGNDFIW

SEQ ID NO: 22353 - protein, 9 aa, synthetic construct
GGSGQDFIF

SEQ ID NO: 22354 - protein, 9 aa, synthetic construct
GGFGNDFLV

SEQ ID NO: 22355 - protein, 9 aa, synthetic construct
GGAGLDNIQ

SEQ ID NO: 22356 - protein, 9 aa, synthetic construct
GGSGQDALT

SEQ ID NO: 22357 - protein, 9 aa, synthetic construct
GGSGQDALM

SEQ ID NO: 22358 - protein, 9 aa, synthetic construct
GGSGQDSLD

SEQ ID NO: 22359 - protein, 9 aa, synthetic construct
GGEGLDRLI

SEQ ID NO: 22360 - protein, 9 aa, synthetic construct
GGSGQDTFS

SEQ ID NO: 22361 - protein, 9 aa, synthetic construct
GGFGNDALT

SEQ ID NO: 22362 - protein, 9 aa, synthetic construct
GGSGRDALY

SEQ ID NO: 22363 - protein, 9 aa, synthetic construct
GGEGLDTLI

SEQ ID NO: 22364 - protein, 9 aa, synthetic construct
GGFGMDTID

SEQ ID NO: 22365 - protein, 9 aa, synthetic construct
GGAGLDDLR

SEQ ID NO: 22366 - protein, 9 aa, synthetic construct
GGSGRDAFK

SEQ ID NO: 22367 - protein, 9 aa, synthetic construct
GGFGMDTLS

SEQ ID NO: 22368 - protein, 9 aa, synthetic construct
GGAGLDDLW

SEQ ID NO: 22369 - protein, 9 aa, synthetic construct
GGSGQDVVD

SEQ ID NO: 22370 - protein, 9 aa, synthetic construct
GGFGNDAIY

SEQ ID NO: 22371 - protein, 9 aa, synthetic construct
GGSGQDVLS

SEQ ID NO: 22372 - protein, 9 aa, synthetic construct
GGSGQDVLI

SEQ ID NO: 22373 - protein, 9 aa, synthetic construct
GGSGQDTYL

SEQ ID NO: 22374 - protein, 9 aa, synthetic construct
GGSGQDTIN

SEQ ID NO: 22375 - protein, 9 aa, synthetic construct
GGSGQDTVY

SEQ ID NO: 22376 - protein, 9 aa, synthetic construct
GGSGQDTVN

SEQ ID NO: 22377 - protein, 9 aa, synthetic construct
GGEGLDSLF

SEQ ID NO: 22378 - protein, 9 aa, synthetic construct
GGSGQDTLM

SEQ ID NO: 22379 - protein, 9 aa, synthetic construct
GGSGQDTLK

SEQ ID NO: 22380 - protein, 9 aa, synthetic construct
GGAGLDHLL

SEQ ID NO: 22381 - protein, 9 aa, synthetic construct
GGSGQDTLF

SEQ ID NO: 22382 - protein, 9 aa, synthetic construct
GGSGQDTLA

SEQ ID NO: 22383 - protein, 9 aa, synthetic construct
GGSGQDTIY

SEQ ID NO: 22384 - protein, 9 aa, synthetic construct
GGAGLDHLY

SEQ ID NO: 22385 - protein, 9 aa, synthetic construct
GGSGQDTIT

SEQ ID NO: 22386 - protein, 9 aa, synthetic construct
GGSGQDALF

SEQ ID NO: 22387 - protein, 9 aa, synthetic construct
GGFGNDHLA

SEQ ID NO: 22388 - protein, 9 aa, synthetic construct
GGSGNDVFH

SEQ ID NO: 22389 - protein, 9 aa, synthetic construct
GGEGLDAAY

SEQ ID NO: 22390 - protein, 9 aa, synthetic construct
GGSGNDWMN

SEQ ID NO: 22391 - protein, 9 aa, synthetic construct
GGEGKDVLR

SEQ ID NO: 22392 - protein, 9 aa, synthetic construct
GGSGNDWLY

SEQ ID NO: 22393 - protein, 9 aa, synthetic construct
GGSGNDWLN

SEQ ID NO: 22394 - protein, 9 aa, synthetic construct
GGSGNDWLI

SEQ ID NO: 22395 - protein, 9 aa, synthetic construct
GGAGLDTAV

SEQ ID NO: 22396 - protein, 9 aa, synthetic construct
GGSGNDWIE

SEQ ID NO: 22397 - protein, 9 aa, synthetic construct
GGSGNDVYY

SEQ ID NO: 22398 - protein, 9 aa, synthetic construct
GGSGNDVYL

SEQ ID NO: 22399 - protein, 9 aa, synthetic construct
GGSGNDVYI

SEQ ID NO: 22400 - protein, 9 aa, synthetic construct
GGSGNDVYF

SEQ ID NO: 22401 - protein, 9 aa, synthetic construct
GGFGNDIYY

SEQ ID NO: 22402 - protein, 9 aa, synthetic construct
GGAGLDTID

SEQ ID NO: 22403 - protein, 9 aa, synthetic construct
GGEGKDVLF

SEQ ID NO: 22404 - protein, 9 aa, synthetic construct
GGFGNDKIQ

SEQ ID NO: 22405 - protein, 9 aa, synthetic construct
GGSGNDVMT

SEQ ID NO: 22406 - protein, 9 aa, synthetic construct
GGSGNDVML

SEQ ID NO: 22407 - protein, 9 aa, synthetic construct
GGSGNDVMI

SEQ ID NO: 22408 - protein, 9 aa, synthetic construct
GGFGNDKLD

SEQ ID NO: 22409 - protein, 9 aa, synthetic construct
GGFGNDKLY

SEQ ID NO: 22410 - protein, 9 aa, synthetic construct
GGSGNDVIM

SEQ ID NO: 22411 - protein, 9 aa, synthetic construct
GGSGNDVIG

SEQ ID NO: 22412 - protein, 9 aa, synthetic construct
GGSGNDVFY

SEQ ID NO: 22413 - protein, 9 aa, synthetic construct
GGSGNDVFR

SEQ ID NO: 22414 - protein, 9 aa, synthetic construct
GGSGNDVFK

SEQ ID NO: 22415 - protein, 9 aa, synthetic construct
GGAGLDSLV

SEQ ID NO: 22416 - protein, 9 aa, synthetic construct
GGAGLDSLT

SEQ ID NO: 22417 - protein, 9 aa, synthetic construct
GGSGNDYID

SEQ ID NO: 22418 - protein, 9 aa, synthetic construct
GGEGKDWFD

SEQ ID NO: 22419 - protein, 9 aa, synthetic construct
GGAGLDQLY

SEQ ID NO: 22420 - protein, 9 aa, synthetic construct
GGAGLDQVR

SEQ ID NO: 22421 - protein, 9 aa, synthetic construct
GGAGLDRID

SEQ ID NO: 22422 - protein, 9 aa, synthetic construct
GGAGLDRIW

SEQ ID NO: 22423 - protein, 9 aa, synthetic construct
GGFGNDIID

SEQ ID NO: 22424 - protein, 9 aa, synthetic construct
GGEGKDYLN

SEQ ID NO: 22425 - protein, 9 aa, synthetic construct
GGAGLDRLL

SEQ ID NO: 22426 - protein, 9 aa, synthetic construct
GGSGPDRFT

SEQ ID NO: 22427 - protein, 9 aa, synthetic construct
GGAGLDRLR

SEQ ID NO: 22428 - protein, 9 aa, synthetic construct
GGAGLDRLT

SEQ ID NO: 22429 - protein, 9 aa, synthetic construct
GGAGLDRMV

SEQ ID NO: 22430 - protein, 9 aa, synthetic construct
GGAGLDSAD

SEQ ID NO: 22431 - protein, 9 aa, synthetic construct
GGAGLDSIS

SEQ ID NO: 22432 - protein, 9 aa, synthetic construct
GGSGNDYVH

SEQ ID NO: 22433 - protein, 9 aa, synthetic construct
GGSGNDYVA

SEQ ID NO: 22434 - protein, 9 aa, synthetic construct
GGFGNDILE

SEQ ID NO: 22435 - protein, 9 aa, synthetic construct
GGSGNDYML

SEQ ID NO: 22436 - protein, 9 aa, synthetic construct
GGAGLDSFI

SEQ ID NO: 22437 - protein, 9 aa, synthetic construct
GGSGNDYLM

SEQ ID NO: 22438 - protein, 9 aa, synthetic construct
GGSGNDYLK

SEQ ID NO: 22439 - protein, 9 aa, synthetic construct
GGFGNDILK

SEQ ID NO: 22440 - protein, 9 aa, synthetic construct
GGSGNDYLF

SEQ ID NO: 22441 - protein, 9 aa, synthetic construct
GGSGNDYIT

SEQ ID NO: 22442 - protein, 9 aa, synthetic construct
GGSGNDYIS

SEQ ID NO: 22443 - protein, 9 aa, synthetic construct
GGSGNDKIN

SEQ ID NO: 22444 - protein, 9 aa, synthetic construct
GGSGNDKIE

SEQ ID NO: 22445 - protein, 9 aa, synthetic construct
GGAGNDHFT

SEQ ID NO: 22446 - protein, 9 aa, synthetic construct
GGSGKDILR

SEQ ID NO: 22447 - protein, 9 aa, synthetic construct
GGAGNDEVF

SEQ ID NO: 22448 - protein, 9 aa, synthetic construct
GGSGKDRLY

SEQ ID NO: 22449 - protein, 9 aa, synthetic construct
GGSGKDRLD

SEQ ID NO: 22450 - protein, 9 aa, synthetic construct
GGSGKDRID

SEQ ID NO: 22451 - protein, 9 aa, synthetic construct
GGSGKDQLS

SEQ ID NO: 22452 - protein, 9 aa, synthetic construct
GGAGNDEVY

SEQ ID NO: 22453 - protein, 9 aa, synthetic construct
GGAGNDEYR

SEQ ID NO: 22454 - protein, 9 aa, synthetic construct
GGFGNDVLI

SEQ ID NO: 22455 - protein, 9 aa, synthetic construct
GGSGKDQFK

SEQ ID NO: 22456 - protein, 9 aa, synthetic construct
GGSGKDQFI

SEQ ID NO: 22457 - protein, 9 aa, synthetic construct
GGEGKDLLF

SEQ ID NO: 22458 - protein, 9 aa, synthetic construct
GGAGNDFFD

SEQ ID NO: 22459 - protein, 9 aa, synthetic construct
GGFGNDVLL

SEQ ID NO: 22460 - protein, 9 aa, synthetic construct
GGSGKDMLF

SEQ ID NO: 22461 - protein, 9 aa, synthetic construct
GGSGKDMLD

SEQ ID NO: 22462 - protein, 9 aa, synthetic construct
GGSGKDMIH

SEQ ID NO: 22463 - protein, 9 aa, synthetic construct
GGSGKDMFV

SEQ ID NO: 22464 - protein, 9 aa, synthetic construct
GGAGNDFFN

SEQ ID NO: 22465 - protein, 9 aa, synthetic construct
GGSGKDLLL

SEQ ID NO: 22466 - protein, 9 aa, synthetic construct
GGSGKDLLD

SEQ ID NO: 22467 - protein, 9 aa, synthetic construct
GGSGKDLIN

SEQ ID NO: 22468 - protein, 9 aa, synthetic construct
GGSGKDKVD

SEQ ID NO: 22469 - protein, 9 aa, synthetic construct
GGAGNDFIG

SEQ ID NO: 22470 - protein, 9 aa, synthetic construct
GGSGKDKFY

SEQ ID NO: 22471 - protein, 9 aa, synthetic construct
GGAGNDFIK

SEQ ID NO: 22472 - protein, 9 aa, synthetic construct
GGSGKDSLD

SEQ ID NO: 22473 - protein, 9 aa, synthetic construct
GGAGNDEML

SEQ ID NO: 22474 - protein, 9 aa, synthetic construct
GGSGKDSYD

SEQ ID NO: 22475 - protein, 9 aa, synthetic construct
GGSGKDVLV

SEQ ID NO: 22476 - protein, 9 aa, synthetic construct
GGSGLDLLR

SEQ ID NO: 22477 - protein, 9 aa, synthetic construct
GGSGLDLLE

SEQ ID NO: 22478 - protein, 9 aa, synthetic construct
GGEGKDNLQ

SEQ ID NO: 22479 - protein, 9 aa, synthetic construct
GGFGNDTYY

SEQ ID NO: 22480 - protein, 9 aa, synthetic construct
GGSGLDIMF

SEQ ID NO: 22481 - protein, 9 aa, synthetic construct
GGFGNDVIF

SEQ ID NO: 22482 - protein, 9 aa, synthetic construct
GGAGNDEIG

SEQ ID NO: 22483 - protein, 9 aa, synthetic construct
GGSGLDFAS

SEQ ID NO: 22484 - protein, 9 aa, synthetic construct
GGSGLDALH

SEQ ID NO: 22485 - protein, 9 aa, synthetic construct
GGSGLDAFR

SEQ ID NO: 22486 - protein, 9 aa, synthetic construct
GGSGKDYFV

SEQ ID NO: 22487 - protein, 9 aa, synthetic construct
GGSGKDVLR

SEQ ID NO: 22488 - protein, 9 aa, synthetic construct
GGSGKDTAS

SEQ ID NO: 22489 - protein, 9 aa, synthetic construct
GGSGKDVLL

SEQ ID NO: 22490 - protein, 9 aa, synthetic construct
GGSGKDVLF

SEQ ID NO: 22491 - protein, 9 aa, synthetic construct
GGSGKDVFD

SEQ ID NO: 22492 - protein, 9 aa, synthetic construct
GGSGKDVFA

SEQ ID NO: 22493 - protein, 9 aa, synthetic construct
GGSGKDTVY

SEQ ID NO: 22494 - protein, 9 aa, synthetic construct
GGSGKDTMT

SEQ ID NO: 22495 - protein, 9 aa, synthetic construct
GGSGKDTLV

SEQ ID NO: 22496 - protein, 9 aa, synthetic construct
GGSGKDTLR

SEQ ID NO: 22497 - protein, 9 aa, synthetic construct
GGSGKDTLK

SEQ ID NO: 22498 - protein, 9 aa, synthetic construct
GGSGKDTLG

SEQ ID NO: 22499 - protein, 9 aa, synthetic construct
GGSGKDTIY

SEQ ID NO: 22500 - protein, 9 aa, synthetic construct
GGSGKDIMY

SEQ ID NO: 22501 - protein, 9 aa, synthetic construct
GGSGKDHLF

SEQ ID NO: 22502 - protein, 9 aa, synthetic construct
GGFGNDTVR

SEQ ID NO: 22503 - protein, 9 aa, synthetic construct
GGSGKDFFV

SEQ ID NO: 22504 - protein, 9 aa, synthetic construct
GGSGIDTAI

SEQ ID NO: 22505 - protein, 9 aa, synthetic construct
GGSGIDTAE

SEQ ID NO: 22506 - protein, 9 aa, synthetic construct
GGSGIDSYD

SEQ ID NO: 22507 - protein, 9 aa, synthetic construct
GGSGIDSMS

SEQ ID NO: 22508 - protein, 9 aa, synthetic construct
GGFGNDYID

SEQ ID NO: 22509 - protein, 9 aa, synthetic construct
GGAGNDGIN

SEQ ID NO: 22510 - protein, 9 aa, synthetic construct
GGEGKDKLI

SEQ ID NO: 22511 - protein, 9 aa, synthetic construct
GGSGIDRLV

SEQ ID NO: 22512 - protein, 9 aa, synthetic construct
GGSGIDRLS

SEQ ID NO: 22513 - protein, 9 aa, synthetic construct
GGFGNDYLE

SEQ ID NO: 22514 - protein, 9 aa, synthetic construct
GGAGNDGLH

SEQ ID NO: 22515 - protein, 9 aa, synthetic construct
GGAGNDGLI

SEQ ID NO: 22516 - protein, 9 aa, synthetic construct
GGSGIDRAS

SEQ ID NO: 22517 - protein, 9 aa, synthetic construct
GGSGIDRAM

SEQ ID NO: 22518 - protein, 9 aa, synthetic construct
GGSGIDQLD

SEQ ID NO: 22519 - protein, 9 aa, synthetic construct
GGAGNDGLV

SEQ ID NO: 22520 - protein, 9 aa, synthetic construct
GGSGIDNLQ

SEQ ID NO: 22521 - protein, 9 aa, synthetic construct
GGSGIDNLM

SEQ ID NO: 22522 - protein, 9 aa, synthetic construct
GGSGIDNLK

SEQ ID NO: 22523 - protein, 9 aa, synthetic construct
GGSGIDMLA

SEQ ID NO: 22524 - protein, 9 aa, synthetic construct
GGAGNDGML

SEQ ID NO: 22525 - protein, 9 aa, synthetic construct
GGAGNDGMV

SEQ ID NO: 22526 - protein, 9 aa, synthetic construct
GGSGIDLLD

SEQ ID NO: 22527 - protein, 9 aa, synthetic construct
GGSGIDLIT

SEQ ID NO: 22528 - protein, 9 aa, synthetic construct
GGSGIDKLY

SEQ ID NO: 22529 - protein, 9 aa, synthetic construct
GGFGNDYIA

SEQ ID NO: 22530 - protein, 9 aa, synthetic construct
GGSGIDTAQ

SEQ ID NO: 22531 - protein, 9 aa, synthetic construct
GGFGNDVYY

SEQ ID NO: 22532 - protein, 9 aa, synthetic construct
GGAGNDFVD

SEQ ID NO: 22533 - protein, 9 aa, synthetic construct
GGSGKDELH

SEQ ID NO: 22534 - protein, 9 aa, synthetic construct
GGSGKDDMW

SEQ ID NO: 22535 - protein, 9 aa, synthetic construct
GGAGNDFLQ

SEQ ID NO: 22536 - protein, 9 aa, synthetic construct
GGSGKDALY

SEQ ID NO: 22537 - protein, 9 aa, synthetic construct
GGSGKDALV

SEQ ID NO: 22538 - protein, 9 aa, synthetic construct
GGSGKDALS

SEQ ID NO: 22539 - protein, 9 aa, synthetic construct
GGSGIDYAS

SEQ ID NO: 22540 - protein, 9 aa, synthetic construct
GGAGNDFMA

SEQ ID NO: 22541 - protein, 9 aa, synthetic construct
GGSGIDVMH

SEQ ID NO: 22542 - protein, 9 aa, synthetic construct
GGAGNDFMG

SEQ ID NO: 22543 - protein, 9 aa, synthetic construct
GGAGNDFMV

SEQ ID NO: 22544 - protein, 9 aa, synthetic construct
GGSGIDTVS

SEQ ID NO: 22545 - protein, 9 aa, synthetic construct
GGFGNDVYV

SEQ ID NO: 22546 - protein, 9 aa, synthetic construct
GGSGIDTVR

SEQ ID NO: 22547 - protein, 9 aa, synthetic construct
GGAGNDFVE

SEQ ID NO: 22548 - protein, 9 aa, synthetic construct
GGSGIDTVI

SEQ ID NO: 22549 - protein, 9 aa, synthetic construct
GGAGNDFVI

SEQ ID NO: 22550 - protein, 9 aa, synthetic construct
GGSGIDTMR

SEQ ID NO: 22551 - protein, 9 aa, synthetic construct
GGEGKDKVR

SEQ ID NO: 22552 - protein, 9 aa, synthetic construct
GGSGIDTLY

SEQ ID NO: 22553 - protein, 9 aa, synthetic construct
GGAGNDFVY

SEQ ID NO: 22554 - protein, 9 aa, synthetic construct
GGSGIDTLH

SEQ ID NO: 22555 - protein, 9 aa, synthetic construct
GGSGIDTLA

SEQ ID NO: 22556 - protein, 9 aa, synthetic construct
GGAGNDFYG

SEQ ID NO: 22557 - protein, 9 aa, synthetic construct
GGFGNDTVS

SEQ ID NO: 22558 - protein, 9 aa, synthetic construct
GGAGNDDVD

SEQ ID NO: 22559 - protein, 9 aa, synthetic construct
GGSGNDIVS

SEQ ID NO: 22560 - protein, 9 aa, synthetic construct
GGAGNDAIQ

SEQ ID NO: 22561 - protein, 9 aa, synthetic construct
GGFGNDTFI

SEQ ID NO: 22562 - protein, 9 aa, synthetic construct
GGSGNDGLF

SEQ ID NO: 22563 - protein, 9 aa, synthetic construct
GGSGNDGLE

SEQ ID NO: 22564 - protein, 9 aa, synthetic construct
GGAGMDVLL

SEQ ID NO: 22565 - protein, 9 aa, synthetic construct
GGSGNDFVT

SEQ ID NO: 22566 - protein, 9 aa, synthetic construct
GGSGNDFVA

SEQ ID NO: 22567 - protein, 9 aa, synthetic construct
GGAGMDWLI

SEQ ID NO: 22568 - protein, 9 aa, synthetic construct
GGSGNDFMS

SEQ ID NO: 22569 - protein, 9 aa, synthetic construct
GGAGMDYAD

SEQ ID NO: 22570 - protein, 9 aa, synthetic construct
GGSGNDFMN

SEQ ID NO: 22571 - protein, 9 aa, synthetic construct
GGSGNDFLT

SEQ ID NO: 22572 - protein, 9 aa, synthetic construct
GGFGNDTII

SEQ ID NO: 22573 - protein, 9 aa, synthetic construct
GGAGNDAAE

SEQ ID NO: 22574 - protein, 9 aa, synthetic construct
GGSGNDFIN

SEQ ID NO: 22575 - protein, 9 aa, synthetic construct
GGAGNDAAG

SEQ ID NO: 22576 - protein, 9 aa, synthetic construct
GGAGNDAAI

SEQ ID NO: 22577 - protein, 9 aa, synthetic construct
GGSGNDFIE

SEQ ID NO: 22578 - protein, 9 aa, synthetic construct
GGAGNDAAN

SEQ ID NO: 22579 - protein, 9 aa, synthetic construct
GGAGNDAAV

SEQ ID NO: 22580 - protein, 9 aa, synthetic construct
GGAGNDAAY

SEQ ID NO: 22581 - protein, 9 aa, synthetic construct
GGSGNDEVY

SEQ ID NO: 22582 - protein, 9 aa, synthetic construct
GGSGNDEVR

SEQ ID NO: 22583 - protein, 9 aa, synthetic construct
GGAGNDAIE

SEQ ID NO: 22584 - protein, 9 aa, synthetic construct
GGSGNDEVA

SEQ ID NO: 22585 - protein, 9 aa, synthetic construct
GGAGNDAIK

SEQ ID NO: 22586 - protein, 9 aa, synthetic construct
GGSGNDGLW

SEQ ID NO: 22587 - protein, 9 aa, synthetic construct
GGEGKDRLF

SEQ ID NO: 22588 - protein, 9 aa, synthetic construct
GGSGNDHAQ

SEQ ID NO: 22589 - protein, 9 aa, synthetic construct
GGSGNDIFK

SEQ ID NO: 22590 - protein, 9 aa, synthetic construct
GGEGKDSVN

SEQ ID NO: 22591 - protein, 9 aa, synthetic construct
GGSGNDIMN

SEQ ID NO: 22592 - protein, 9 aa, synthetic construct
GGAGMDTAS

SEQ ID NO: 22593 - protein, 9 aa, synthetic construct
GGAGMDTAV

SEQ ID NO: 22594 - protein, 9 aa, synthetic construct
GGAGMDTAY

SEQ ID NO: 22595 - protein, 9 aa, synthetic construct
GGSGNDIIQ

SEQ ID NO: 22596 - protein, 9 aa, synthetic construct
GGAGMDTFV

SEQ ID NO: 22597 - protein, 9 aa, synthetic construct
GGFGNDSLR

SEQ ID NO: 22598 - protein, 9 aa, synthetic construct
GGAGMDTID

SEQ ID NO: 22599 - protein, 9 aa, synthetic construct
GGSGNDIFS

SEQ ID NO: 22600 - protein, 9 aa, synthetic construct
GGSGNDIFL

SEQ ID NO: 22601 - protein, 9 aa, synthetic construct
GGSGNDIFI

SEQ ID NO: 22602 - protein, 9 aa, synthetic construct
GGAGMDTYV

SEQ ID NO: 22603 - protein, 9 aa, synthetic construct
GGFGNDSMR

SEQ ID NO: 22604 - protein, 9 aa, synthetic construct
GGSGNDIAY

SEQ ID NO: 22605 - protein, 9 aa, synthetic construct
GGSGNDIAL

SEQ ID NO: 22606 - protein, 9 aa, synthetic construct
GGFGNDSVF

SEQ ID NO: 22607 - protein, 9 aa, synthetic construct
GGSGNDHML

SEQ ID NO: 22608 - protein, 9 aa, synthetic construct
GGSGNDHLW

SEQ ID NO: 22609 - protein, 9 aa, synthetic construct
GGAGMDTLV

SEQ ID NO: 22610 - protein, 9 aa, synthetic construct
GGAGMDTLY

SEQ ID NO: 22611 - protein, 9 aa, synthetic construct
GGSGNDHID

SEQ ID NO: 22612 - protein, 9 aa, synthetic construct
GGFGNDSYV

SEQ ID NO: 22613 - protein, 9 aa, synthetic construct
GGSGNDHFV

SEQ ID NO: 22614 - protein, 9 aa, synthetic construct
GGSGNDEMN

SEQ ID NO: 22615 - protein, 9 aa, synthetic construct
GGSGNDELW

SEQ ID NO: 22616 - protein, 9 aa, synthetic construct
GGAGNDDMY

SEQ ID NO: 22617 - protein, 9 aa, synthetic construct
GGSGNDELN

SEQ ID NO: 22618 - protein, 9 aa, synthetic construct
GGAGNDDIV

SEQ ID NO: 22619 - protein, 9 aa, synthetic construct
GGAGNDDIY

SEQ ID NO: 22620 - protein, 9 aa, synthetic construct
GGSGLDVLS

SEQ ID NO: 22621 - protein, 9 aa, synthetic construct
GGSGLDVLD

SEQ ID NO: 22622 - protein, 9 aa, synthetic construct
GGSGLDVIL

SEQ ID NO: 22623 - protein, 9 aa, synthetic construct
GGEGKDQLY

SEQ ID NO: 22624 - protein, 9 aa, synthetic construct
GGAGNDDLN

SEQ ID NO: 22625 - protein, 9 aa, synthetic construct
GGSGLDTLV

SEQ ID NO: 22626 - protein, 9 aa, synthetic construct
GGSGLDTLT

SEQ ID NO: 22627 - protein, 9 aa, synthetic construct
GGSGLDTLN

SEQ ID NO: 22628 - protein, 9 aa, synthetic construct
GGSGLDTLD

SEQ ID NO: 22629 - protein, 9 aa, synthetic construct
GGSGLDTLA

SEQ ID NO: 22630 - protein, 9 aa, synthetic construct
GGSGLDTIY

SEQ ID NO: 22631 - protein, 9 aa, synthetic construct
GGAGNDDLW

SEQ ID NO: 22632 - protein, 9 aa, synthetic construct
GGFGNDTMS

SEQ ID NO: 22633 - protein, 9 aa, synthetic construct
GGSGLDTAR

SEQ ID NO: 22634 - protein, 9 aa, synthetic construct
GGSGLDTAD

SEQ ID NO: 22635 - protein, 9 aa, synthetic construct
GGSGLDSLS

SEQ ID NO: 22636 - protein, 9 aa, synthetic construct
GGSGLDSLF

SEQ ID NO: 22637 - protein, 9 aa, synthetic construct
GGAGNDDMF

SEQ ID NO: 22638 - protein, 9 aa, synthetic construct
GGSGLDRVI

SEQ ID NO: 22639 - protein, 9 aa, synthetic construct
GGSGLDRLV

SEQ ID NO: 22640 - protein, 9 aa, synthetic construct
GGSGLDRLQ

SEQ ID NO: 22641 - protein, 9 aa, synthetic construct
GGSGLDRLE

SEQ ID NO: 22642 - protein, 9 aa, synthetic construct
GGSGLDRAQ

SEQ ID NO: 22643 - protein, 9 aa, synthetic construct
GGAGNDDIL

SEQ ID NO: 22644 - protein, 9 aa, synthetic construct
GGAGNDDIG

SEQ ID NO: 22645 - protein, 9 aa, synthetic construct
GGSGMDILE

SEQ ID NO: 22646 - protein, 9 aa, synthetic construct
GGSGNDALL

SEQ ID NO: 22647 - protein, 9 aa, synthetic construct
GGSGNDELF

SEQ ID NO: 22648 - protein, 9 aa, synthetic construct
GGSGNDEIW

SEQ ID NO: 22649 - protein, 9 aa, synthetic construct
GGSGNDEIA

SEQ ID NO: 22650 - protein, 9 aa, synthetic construct
GGSGNDDLV

SEQ ID NO: 22651 - protein, 9 aa, synthetic construct
GGSGNDDIT

SEQ ID NO: 22652 - protein, 9 aa, synthetic construct
GGAGNDAMA

SEQ ID NO: 22653 - protein, 9 aa, synthetic construct
GGAGNDAMF

SEQ ID NO: 22654 - protein, 9 aa, synthetic construct
GGAGNDAMS

SEQ ID NO: 22655 - protein, 9 aa, synthetic construct
GGAGNDAMY

SEQ ID NO: 22656 - protein, 9 aa, synthetic construct
GGSGNDAMF

SEQ ID NO: 22657 - protein, 9 aa, synthetic construct
GGSGNDALW

SEQ ID NO: 22658 - protein, 9 aa, synthetic construct
GGSGNDALK

SEQ ID NO: 22659 - protein, 9 aa, synthetic construct
GGSGMDILI

SEQ ID NO: 22660 - protein, 9 aa, synthetic construct
GGSGNDALE

SEQ ID NO: 22661 - protein, 9 aa, synthetic construct
GGAGNDAVT

SEQ ID NO: 22662 - protein, 9 aa, synthetic construct
GGSGNDAFY

SEQ ID NO: 22663 - protein, 9 aa, synthetic construct
GGAGNDAYL

SEQ ID NO: 22664 - protein, 9 aa, synthetic construct
GGSGMDTLY

SEQ ID NO: 22665 - protein, 9 aa, synthetic construct
GGSGMDTLI

SEQ ID NO: 22666 - protein, 9 aa, synthetic construct
GGSGMDTIW

SEQ ID NO: 22667 - protein, 9 aa, synthetic construct
GGEGKDRIL

SEQ ID NO: 22668 - protein, 9 aa, synthetic construct
GGSGMDRLF

SEQ ID NO: 22669 - protein, 9 aa, synthetic construct
GGAGNDDFL

SEQ ID NO: 22670 - protein, 9 aa, synthetic construct
GGAGNDDFT

SEQ ID NO: 22671 - protein, 9 aa, synthetic construct
GGTGGDTLY

SEQ ID NO: 22672 - protein, 9 aa, synthetic construct
GGFGADILN

SEQ ID NO: 22673 - protein, 9 aa, synthetic construct
GGFGADILL

SEQ ID NO: 22674 - protein, 9 aa, synthetic construct
GGAGDDDLL

SEQ ID NO: 22675 - protein, 9 aa, synthetic construct
GGVGNDTVT

SEQ ID NO: 22676 - protein, 9 aa, synthetic construct
GGVGNDTML

SEQ ID NO: 22677 - protein, 9 aa, synthetic construct
GGVGNDTLH

SEQ ID NO: 22678 - protein, 9 aa, synthetic construct
GGAGDDDMF

SEQ ID NO: 22679 - protein, 9 aa, synthetic construct
GGVGNDTIR

SEQ ID NO: 22680 - protein, 9 aa, synthetic construct
GGVGNDTIQ

SEQ ID NO: 22681 - protein, 9 aa, synthetic construct
GGVGNDTIN

SEQ ID NO: 22682 - protein, 9 aa, synthetic construct
GGEGSDEIS

SEQ ID NO: 22683 - protein, 9 aa, synthetic construct
GGVGNDTIH

SEQ ID NO: 22684 - protein, 9 aa, synthetic construct
GGVGNDTIE

SEQ ID NO: 22685 - protein, 9 aa, synthetic construct
GGVGNDTFY

SEQ ID NO: 22686 - protein, 9 aa, synthetic construct
GGVGNDTFQ

SEQ ID NO: 22687 - protein, 9 aa, synthetic construct
GGVGNDTFL

SEQ ID NO: 22688 - protein, 9 aa, synthetic construct
GGEGSDEIT

SEQ ID NO: 22689 - protein, 9 aa, synthetic construct
GGEGSDEIY

SEQ ID NO: 22690 - protein, 9 aa, synthetic construct
GGEGSDELD

SEQ ID NO: 22691 - protein, 9 aa, synthetic construct
GGVGNDTAS

SEQ ID NO: 22692 - protein, 9 aa, synthetic construct
GGVGNDTAR

SEQ ID NO: 22693 - protein, 9 aa, synthetic construct
GGAGDDDYV

SEQ ID NO: 22694 - protein, 9 aa, synthetic construct
GGAGDDEAQ

SEQ ID NO: 22695 - protein, 9 aa, synthetic construct
GGEGSDELY

SEQ ID NO: 22696 - protein, 9 aa, synthetic construct
GGVGNDSMH

SEQ ID NO: 22697 - protein, 9 aa, synthetic construct
GGAGDDEIF

SEQ ID NO: 22698 - protein, 9 aa, synthetic construct
GGVGNDSLI

SEQ ID NO: 22699 - protein, 9 aa, synthetic construct
GGVGNDRYE

SEQ ID NO: 22700 - protein, 9 aa, synthetic construct
GGAGDDDLQ

SEQ ID NO: 22701 - protein, 9 aa, synthetic construct
GGVGNDVAV

SEQ ID NO: 22702 - protein, 9 aa, synthetic construct
GGVGADVFR

SEQ ID NO: 22703 - protein, 9 aa, synthetic construct
GGVGNDVAY

SEQ ID NO: 22704 - protein, 9 aa, synthetic construct
GGAGDDAMT

SEQ ID NO: 22705 - protein, 9 aa, synthetic construct
GGEGSDALE

SEQ ID NO: 22706 - protein, 9 aa, synthetic construct
GGVGQDEFV

SEQ ID NO: 22707 - protein, 9 aa, synthetic construct
GGVGPDYLE

SEQ ID NO: 22708 - protein, 9 aa, synthetic construct
GGVGPDTLS

SEQ ID NO: 22709 - protein, 9 aa, synthetic construct
GGEGSDALY

SEQ ID NO: 22710 - protein, 9 aa, synthetic construct
GGAGDDAVS

SEQ ID NO: 22711 - protein, 9 aa, synthetic construct
GGAGDDAVY

SEQ ID NO: 22712 - protein, 9 aa, synthetic construct
GGVGPDKFV

SEQ ID NO: 22713 - protein, 9 aa, synthetic construct
GGEGSDAVH

SEQ ID NO: 22714 - protein, 9 aa, synthetic construct
GGVGNDYMA

SEQ ID NO: 22715 - protein, 9 aa, synthetic construct
GGVGNDYIF

SEQ ID NO: 22716 - protein, 9 aa, synthetic construct
GGAGDDCLR

SEQ ID NO: 22717 - protein, 9 aa, synthetic construct
GGVGNDYFY

SEQ ID NO: 22718 - protein, 9 aa, synthetic construct
GGVGNDYAS

SEQ ID NO: 22719 - protein, 9 aa, synthetic construct
GGAGDDCMA

SEQ ID NO: 22720 - protein, 9 aa, synthetic construct
GGVGNDWID

SEQ ID NO: 22721 - protein, 9 aa, synthetic construct
GGVGNDVYV

SEQ ID NO: 22722 - protein, 9 aa, synthetic construct
GGVGNDVYL

SEQ ID NO: 22723 - protein, 9 aa, synthetic construct
GGAGDDDIG

SEQ ID NO: 22724 - protein, 9 aa, synthetic construct
GGVGNDVMV

SEQ ID NO: 22725 - protein, 9 aa, synthetic construct
GGVGNDVLY

SEQ ID NO: 22726 - protein, 9 aa, synthetic construct
GGVGNDVLM

SEQ ID NO: 22727 - protein, 9 aa, synthetic construct
GGVGNDVII

SEQ ID NO: 22728 - protein, 9 aa, synthetic construct
GGVGNDVID

SEQ ID NO: 22729 - protein, 9 aa, synthetic construct
GGAGDDEIQ

SEQ ID NO: 22730 - protein, 9 aa, synthetic construct
GGVGNDRMV

SEQ ID NO: 22731 - protein, 9 aa, synthetic construct
GGVGNDRLG

SEQ ID NO: 22732 - protein, 9 aa, synthetic construct
GGVGNDRLA

SEQ ID NO: 22733 - protein, 9 aa, synthetic construct
GGAGDDFFI

SEQ ID NO: 22734 - protein, 9 aa, synthetic construct
GGEGNDVFK

SEQ ID NO: 22735 - protein, 9 aa, synthetic construct
GGVGNDLLE

SEQ ID NO: 22736 - protein, 9 aa, synthetic construct
GGVGNDLLA

SEQ ID NO: 22737 - protein, 9 aa, synthetic construct
GGVGNDLIT

SEQ ID NO: 22738 - protein, 9 aa, synthetic construct
GGAGDDFIE

SEQ ID NO: 22739 - protein, 9 aa, synthetic construct
GGAGDDFIG

SEQ ID NO: 22740 - protein, 9 aa, synthetic construct
GGVGNDLIE

SEQ ID NO: 22741 - protein, 9 aa, synthetic construct
GGAGDDFII

SEQ ID NO: 22742 - protein, 9 aa, synthetic construct
GGAGDDFIL

SEQ ID NO: 22743 - protein, 9 aa, synthetic construct
GGAGDDFIV

SEQ ID NO: 22744 - protein, 9 aa, synthetic construct
GGVGNDIYF

SEQ ID NO: 22745 - protein, 9 aa, synthetic construct
GGVGNDIVV

SEQ ID NO: 22746 - protein, 9 aa, synthetic construct
GGVGNDIVK

SEQ ID NO: 22747 - protein, 9 aa, synthetic construct
GGVGNDILQ

SEQ ID NO: 22748 - protein, 9 aa, synthetic construct
GGVGNDILK

SEQ ID NO: 22749 - protein, 9 aa, synthetic construct
GGVGNDILE

SEQ ID NO: 22750 - protein, 9 aa, synthetic construct
GGVGNDIIT

SEQ ID NO: 22751 - protein, 9 aa, synthetic construct
GGVGNDIFV

SEQ ID NO: 22752 - protein, 9 aa, synthetic construct
GGVGNDIFD

SEQ ID NO: 22753 - protein, 9 aa, synthetic construct
GGVGNDHLQ

SEQ ID NO: 22754 - protein, 9 aa, synthetic construct
GGVGNDHLN

SEQ ID NO: 22755 - protein, 9 aa, synthetic construct
GGVGNDHLE

SEQ ID NO: 22756 - protein, 9 aa, synthetic construct
GGEGNDVFD

SEQ ID NO: 22757 - protein, 9 aa, synthetic construct
GGEGNDVAS

SEQ ID NO: 22758 - protein, 9 aa, synthetic construct
GGVGNDLVF

SEQ ID NO: 22759 - protein, 9 aa, synthetic construct
GGEGNDVFS

SEQ ID NO: 22760 - protein, 9 aa, synthetic construct
GGAGDDEYY

SEQ ID NO: 22761 - protein, 9 aa, synthetic construct
GGAGDDEMW

SEQ ID NO: 22762 - protein, 9 aa, synthetic construct
GGVGNDRIS

SEQ ID NO: 22763 - protein, 9 aa, synthetic construct
GGVGNDRIR

SEQ ID NO: 22764 - protein, 9 aa, synthetic construct
GGVGNDRID

SEQ ID NO: 22765 - protein, 9 aa, synthetic construct
GGVGNDQLT

SEQ ID NO: 22766 - protein, 9 aa, synthetic construct
GGEGSDFLT

SEQ ID NO: 22767 - protein, 9 aa, synthetic construct
GGAGDDEMH

SEQ ID NO: 22768 - protein, 9 aa, synthetic construct
GGVGNDQLK

SEQ ID NO: 22769 - protein, 9 aa, synthetic construct
GGAGDDEMI

SEQ ID NO: 22770 - protein, 9 aa, synthetic construct
GGAGDDEMN

SEQ ID NO: 22771 - protein, 9 aa, synthetic construct
GGVGNDQLD

SEQ ID NO: 22772 - protein, 9 aa, synthetic construct
GGAGDDEMR

SEQ ID NO: 22773 - protein, 9 aa, synthetic construct
GGEGNDVIR

SEQ ID NO: 22774 - protein, 9 aa, synthetic construct
GGVGNDLYI

SEQ ID NO: 22775 - protein, 9 aa, synthetic construct
GGAGDDEVH

SEQ ID NO: 22776 - protein, 9 aa, synthetic construct
GGEGSDHIE

SEQ ID NO: 22777 - protein, 9 aa, synthetic construct
GGEGNDVIG

SEQ ID NO: 22778 - protein, 9 aa, synthetic construct
GGVGNDNLQ

SEQ ID NO: 22779 - protein, 9 aa, synthetic construct
GGEGSDHLV

SEQ ID NO: 22780 - protein, 9 aa, synthetic construct
GGVGNDNIT

SEQ ID NO: 22781 - protein, 9 aa, synthetic construct
GGVGNDMLW

SEQ ID NO: 22782 - protein, 9 aa, synthetic construct
GGAGDDEYV

SEQ ID NO: 22783 - protein, 9 aa, synthetic construct
GGVGNDMID

SEQ ID NO: 22784 - protein, 9 aa, synthetic construct
GGVGNDLYV

SEQ ID NO: 22785 - protein, 9 aa, synthetic construct
GGVGNDLYL

SEQ ID NO: 22786 - protein, 9 aa, synthetic construct
GGVGQDHLL

SEQ ID NO: 22787 - protein, 9 aa, synthetic construct
GGVGQDIFV

SEQ ID NO: 22788 - protein, 9 aa, synthetic construct
GGVGQDRIS

SEQ ID NO: 22789 - protein, 9 aa, synthetic construct
GGVGSDQLF

SEQ ID NO: 22790 - protein, 9 aa, synthetic construct
GGAGADVMH

SEQ ID NO: 22791 - protein, 9 aa, synthetic construct
GGVGTDIMT

SEQ ID NO: 22792 - protein, 9 aa, synthetic construct
GGVGTDILV

SEQ ID NO: 22793 - protein, 9 aa, synthetic construct
GGVGTDILT

SEQ ID NO: 22794 - protein, 9 aa, synthetic construct
GGVGTDHLY

SEQ ID NO: 22795 - protein, 9 aa, synthetic construct
GGAGADVVD

SEQ ID NO: 22796 - protein, 9 aa, synthetic construct
GGAGADVVV

SEQ ID NO: 22797 - protein, 9 aa, synthetic construct
GGVGSDVLT

SEQ ID NO: 22798 - protein, 9 aa, synthetic construct
GGVGSDVFR

SEQ ID NO: 22799 - protein, 9 aa, synthetic construct
GGAGADVYR

SEQ ID NO: 22800 - protein, 9 aa, synthetic construct
GGVGSDTYL

SEQ ID NO: 22801 - protein, 9 aa, synthetic construct
GGVGSDTVV

SEQ ID NO: 22802 - protein, 9 aa, synthetic construct
GGVGSDTLL

SEQ ID NO: 22803 - protein, 9 aa, synthetic construct
GGEGRDTMF

SEQ ID NO: 22804 - protein, 9 aa, synthetic construct
GGVGSDTII

SEQ ID NO: 22805 - protein, 9 aa, synthetic construct
GGAGADWFY

SEQ ID NO: 22806 - protein, 9 aa, synthetic construct
GGVGSDTIF

SEQ ID NO: 22807 - protein, 9 aa, synthetic construct
GGAGADWIS

SEQ ID NO: 22808 - protein, 9 aa, synthetic construct
GGAGADWLA

SEQ ID NO: 22809 - protein, 9 aa, synthetic construct
GGVGSDSLS

SEQ ID NO: 22810 - protein, 9 aa, synthetic construct
GGAGADWLH

SEQ ID NO: 22811 - protein, 9 aa, synthetic construct
GGVGSDSAS

SEQ ID NO: 22812 - protein, 9 aa, synthetic construct
GGAGADWLL

SEQ ID NO: 22813 - protein, 9 aa, synthetic construct
GGVGSDRLI

SEQ ID NO: 22814 - protein, 9 aa, synthetic construct
GGAGADWLV

SEQ ID NO: 22815 - protein, 9 aa, synthetic construct
GGVGTDLAS

SEQ ID NO: 22816 - protein, 9 aa, synthetic construct
GGAGADVME

SEQ ID NO: 22817 - protein, 9 aa, synthetic construct
GGVGTDNLV

SEQ ID NO: 22818 - protein, 9 aa, synthetic construct
GGVGTDTLS

SEQ ID NO: 22819 - protein, 9 aa, synthetic construct
GGVGVDRLT

SEQ ID NO: 22820 - protein, 9 aa, synthetic construct
GGAGADVFS

SEQ ID NO: 22821 - protein, 9 aa, synthetic construct
GGAGADVFW

SEQ ID NO: 22822 - protein, 9 aa, synthetic construct
GGAGADVFY

SEQ ID NO: 22823 - protein, 9 aa, synthetic construct
GGVGVDQLN

SEQ ID NO: 22824 - protein, 9 aa, synthetic construct
GGEGRDTLK

SEQ ID NO: 22825 - protein, 9 aa, synthetic construct
GGVGVDHFD

SEQ ID NO: 22826 - protein, 9 aa, synthetic construct
GGAGADVIQ

SEQ ID NO: 22827 - protein, 9 aa, synthetic construct
GGVGTDVMA

SEQ ID NO: 22828 - protein, 9 aa, synthetic construct
GGVGTDVLR

SEQ ID NO: 22829 - protein, 9 aa, synthetic construct
GGVGTDTLY

SEQ ID NO: 22830 - protein, 9 aa, synthetic construct
GGVGTDTLQ

SEQ ID NO: 22831 - protein, 9 aa, synthetic construct
GGVGTDRLS

SEQ ID NO: 22832 - protein, 9 aa, synthetic construct
GGVGTDTLL

SEQ ID NO: 22833 - protein, 9 aa, synthetic construct
GGVGTDTIT

SEQ ID NO: 22834 - protein, 9 aa, synthetic construct
GGVGTDTAV

SEQ ID NO: 22835 - protein, 9 aa, synthetic construct
GGVGTDTAD

SEQ ID NO: 22836 - protein, 9 aa, synthetic construct
GGVGTDSMT

SEQ ID NO: 22837 - protein, 9 aa, synthetic construct
GGVGTDSLT

SEQ ID NO: 22838 - protein, 9 aa, synthetic construct
GGVGTDSLL

SEQ ID NO: 22839 - protein, 9 aa, synthetic construct
GGVGTDSLD

SEQ ID NO: 22840 - protein, 9 aa, synthetic construct
GGVGTDRMS

SEQ ID NO: 22841 - protein, 9 aa, synthetic construct
GGVGTDRLY

SEQ ID NO: 22842 - protein, 9 aa, synthetic construct
GGVGTDRLT

SEQ ID NO: 22843 - protein, 9 aa, synthetic construct
GGVGSDQMW

SEQ ID NO: 22844 - protein, 9 aa, synthetic construct
GGVGSDLLS

SEQ ID NO: 22845 - protein, 9 aa, synthetic construct
GGAGDDALM

SEQ ID NO: 22846 - protein, 9 aa, synthetic construct
GGEGRDVFN

SEQ ID NO: 22847 - protein, 9 aa, synthetic construct
GGVGRDSLL

SEQ ID NO: 22848 - protein, 9 aa, synthetic construct
GGEGRDVML

SEQ ID NO: 22849 - protein, 9 aa, synthetic construct
GGVGRDRLF

SEQ ID NO: 22850 - protein, 9 aa, synthetic construct
GGVGRDRID

SEQ ID NO: 22851 - protein, 9 aa, synthetic construct
GGAGCDRLV

SEQ ID NO: 22852 - protein, 9 aa, synthetic construct
GGEGRDVVR

SEQ ID NO: 22853 - protein, 9 aa, synthetic construct
GGEGNDVML

SEQ ID NO: 22854 - protein, 9 aa, synthetic construct
GGEGRDWLE

SEQ ID NO: 22855 - protein, 9 aa, synthetic construct
GGAGDDAAL

SEQ ID NO: 22856 - protein, 9 aa, synthetic construct
GGVGRDKMI

SEQ ID NO: 22857 - protein, 9 aa, synthetic construct
GGVGRDKLL

SEQ ID NO: 22858 - protein, 9 aa, synthetic construct
GGAGDDAFD

SEQ ID NO: 22859 - protein, 9 aa, synthetic construct
GGVGRDILL

SEQ ID NO: 22860 - protein, 9 aa, synthetic construct
GGVGRDFLS

SEQ ID NO: 22861 - protein, 9 aa, synthetic construct
GGVGRDDMT

SEQ ID NO: 22862 - protein, 9 aa, synthetic construct
GGAGDDAIH

SEQ ID NO: 22863 - protein, 9 aa, synthetic construct
GGAGDDAIN

SEQ ID NO: 22864 - protein, 9 aa, synthetic construct
GGEGSDAIF

SEQ ID NO: 22865 - protein, 9 aa, synthetic construct
GGAGDDAIT

SEQ ID NO: 22866 - protein, 9 aa, synthetic construct
GGVGQDVFV

SEQ ID NO: 22867 - protein, 9 aa, synthetic construct
GGVGQDVFR

SEQ ID NO: 22868 - protein, 9 aa, synthetic construct
GGVGQDTLY

SEQ ID NO: 22869 - protein, 9 aa, synthetic construct
GGVGQDTLN

SEQ ID NO: 22870 - protein, 9 aa, synthetic construct
GGVGQDTLK

SEQ ID NO: 22871 - protein, 9 aa, synthetic construct
GGAGDDALG

SEQ ID NO: 22872 - protein, 9 aa, synthetic construct
GGAGADYVR

SEQ ID NO: 22873 - protein, 9 aa, synthetic construct
GGEGRDVLV

SEQ ID NO: 22874 - protein, 9 aa, synthetic construct
GGVGRDTIT

SEQ ID NO: 22875 - protein, 9 aa, synthetic construct
GGAGADYIY

SEQ ID NO: 22876 - protein, 9 aa, synthetic construct
GGVGSDLLQ

SEQ ID NO: 22877 - protein, 9 aa, synthetic construct
GGVGSDLLD

SEQ ID NO: 22878 - protein, 9 aa, synthetic construct
GGEGRDVID

SEQ ID NO: 22879 - protein, 9 aa, synthetic construct
GGVGSDLFL

SEQ ID NO: 22880 - protein, 9 aa, synthetic construct
GGEGNDVVQ

SEQ ID NO: 22881 - protein, 9 aa, synthetic construct
GGVGSDKME

SEQ ID NO: 22882 - protein, 9 aa, synthetic construct
GGEGRDVIY

SEQ ID NO: 22883 - protein, 9 aa, synthetic construct
GGVGSDIVR

SEQ ID NO: 22884 - protein, 9 aa, synthetic construct
GGVGSDILS

SEQ ID NO: 22885 - protein, 9 aa, synthetic construct
GGVGSDILN

SEQ ID NO: 22886 - protein, 9 aa, synthetic construct
GGAGADYIV

SEQ ID NO: 22887 - protein, 9 aa, synthetic construct
GGAGADYLH

SEQ ID NO: 22888 - protein, 9 aa, synthetic construct
GGVGRDTLD

SEQ ID NO: 22889 - protein, 9 aa, synthetic construct
GGVGSDFIH

SEQ ID NO: 22890 - protein, 9 aa, synthetic construct
GGVGSDDLA

SEQ ID NO: 22891 - protein, 9 aa, synthetic construct
GGVGSDALF

SEQ ID NO: 22892 - protein, 9 aa, synthetic construct
GGAGADYMF

SEQ ID NO: 22893 - protein, 9 aa, synthetic construct
GGVGRDVVF

SEQ ID NO: 22894 - protein, 9 aa, synthetic construct
GGAGADYMI

SEQ ID NO: 22895 - protein, 9 aa, synthetic construct
GGAGADYMN

SEQ ID NO: 22896 - protein, 9 aa, synthetic construct
GGVGRDTVR

SEQ ID NO: 22897 - protein, 9 aa, synthetic construct
GGVGRDTLR

SEQ ID NO: 22898 - protein, 9 aa, synthetic construct
GGAGADYMV

SEQ ID NO: 22899 - protein, 9 aa, synthetic construct
GGVGRDTLE

SEQ ID NO: 22900 - protein, 9 aa, synthetic construct
GGVGNDGLS

SEQ ID NO: 22901 - protein, 9 aa, synthetic construct
GGVGNDGLN

SEQ ID NO: 22902 - protein, 9 aa, synthetic construct
GGVGNDGLA

SEQ ID NO: 22903 - protein, 9 aa, synthetic construct
GGVGDDQLT

SEQ ID NO: 22904 - protein, 9 aa, synthetic construct
GGVGDDTYR

SEQ ID NO: 22905 - protein, 9 aa, synthetic construct
GGVGDDTVE

SEQ ID NO: 22906 - protein, 9 aa, synthetic construct
GGVGDDTVD

SEQ ID NO: 22907 - protein, 9 aa, synthetic construct
GGVGDDTMY

SEQ ID NO: 22908 - protein, 9 aa, synthetic construct
GGVGDDTMT

SEQ ID NO: 22909 - protein, 9 aa, synthetic construct
GGVGDDTML

SEQ ID NO: 22910 - protein, 9 aa, synthetic construct
GGVGDDTLW

SEQ ID NO: 22911 - protein, 9 aa, synthetic construct
GGVGDDTLM

SEQ ID NO: 22912 - protein, 9 aa, synthetic construct
GGVGDDTLH

SEQ ID NO: 22913 - protein, 9 aa, synthetic construct
GGVGDDTIY

SEQ ID NO: 22914 - protein, 9 aa, synthetic construct
GGVGDDTIL

SEQ ID NO: 22915 - protein, 9 aa, synthetic construct
GGVGDDTIF

SEQ ID NO: 22916 - protein, 9 aa, synthetic construct
GGVGDDTFV

SEQ ID NO: 22917 - protein, 9 aa, synthetic construct
GGAGDDLIT

SEQ ID NO: 22918 - protein, 9 aa, synthetic construct
GGAGDDLIW

SEQ ID NO: 22919 - protein, 9 aa, synthetic construct
GGVGDDTAT

SEQ ID NO: 22920 - protein, 9 aa, synthetic construct
GGVGDDSYQ

SEQ ID NO: 22921 - protein, 9 aa, synthetic construct
GGVGDDSVS

SEQ ID NO: 22922 - protein, 9 aa, synthetic construct
GGVGDDSLG

SEQ ID NO: 22923 - protein, 9 aa, synthetic construct
GGVGDDSIE

SEQ ID NO: 22924 - protein, 9 aa, synthetic construct
GGAGDDLMD

SEQ ID NO: 22925 - protein, 9 aa, synthetic construct
GGAGDDLMH

SEQ ID NO: 22926 - protein, 9 aa, synthetic construct
GGVGDDRLE

SEQ ID NO: 22927 - protein, 9 aa, synthetic construct
GGAGDDLMQ

SEQ ID NO: 22928 - protein, 9 aa, synthetic construct
GGVGDDRAF

SEQ ID NO: 22929 - protein, 9 aa, synthetic construct
GGVGDDVFL

SEQ ID NO: 22930 - protein, 9 aa, synthetic construct
GGVGDDVID

SEQ ID NO: 22931 - protein, 9 aa, synthetic construct
GGVGDDVMV

SEQ ID NO: 22932 - protein, 9 aa, synthetic construct
GGAGDDKVM

SEQ ID NO: 22933 - protein, 9 aa, synthetic construct
GGVGEDTIN

SEQ ID NO: 22934 - protein, 9 aa, synthetic construct
GGVGEDRLH

SEQ ID NO: 22935 - protein, 9 aa, synthetic construct
GGVGEDRLF

SEQ ID NO: 22936 - protein, 9 aa, synthetic construct
GGVGEDQLF

SEQ ID NO: 22937 - protein, 9 aa, synthetic construct
GGVGEDLMK

SEQ ID NO: 22938 - protein, 9 aa, synthetic construct
GGEGSDNID

SEQ ID NO: 22939 - protein, 9 aa, synthetic construct
GGVGEDLFL

SEQ ID NO: 22940 - protein, 9 aa, synthetic construct
GGVGEDKLR

SEQ ID NO: 22941 - protein, 9 aa, synthetic construct
GGAGDDKMY

SEQ ID NO: 22942 - protein, 9 aa, synthetic construct
GGVGEDIIY

SEQ ID NO: 22943 - protein, 9 aa, synthetic construct
GGAGDDKVL

SEQ ID NO: 22944 - protein, 9 aa, synthetic construct
GGVGEDCFV

SEQ ID NO: 22945 - protein, 9 aa, synthetic construct
GGVGDDVVR

SEQ ID NO: 22946 - protein, 9 aa, synthetic construct
GGVGDDYMY

SEQ ID NO: 22947 - protein, 9 aa, synthetic construct
GGAGDDKYY

SEQ ID NO: 22948 - protein, 9 aa, synthetic construct
GGAGDDLAE

SEQ ID NO: 22949 - protein, 9 aa, synthetic construct
GGEGSDNVD

SEQ ID NO: 22950 - protein, 9 aa, synthetic construct
GGAGDDLAH

SEQ ID NO: 22951 - protein, 9 aa, synthetic construct
GGAGDDLAR

SEQ ID NO: 22952 - protein, 9 aa, synthetic construct
GGVGDDWLY

SEQ ID NO: 22953 - protein, 9 aa, synthetic construct
GGVGDDWLI

SEQ ID NO: 22954 - protein, 9 aa, synthetic construct
GGVGDDVYR

SEQ ID NO: 22955 - protein, 9 aa, synthetic construct
GGVGDDVVT

SEQ ID NO: 22956 - protein, 9 aa, synthetic construct
GGVGDDVVS

SEQ ID NO: 22957 - protein, 9 aa, synthetic construct
GGEGSDRFF

SEQ ID NO: 22958 - protein, 9 aa, synthetic construct
GGVGDDQIN

SEQ ID NO: 22959 - protein, 9 aa, synthetic construct
GGVGEDVLR

SEQ ID NO: 22960 - protein, 9 aa, synthetic construct
GGAGDDLVK

SEQ ID NO: 22961 - protein, 9 aa, synthetic construct
GGVGDDELD

SEQ ID NO: 22962 - protein, 9 aa, synthetic construct
GGAGDDMYF

SEQ ID NO: 22963 - protein, 9 aa, synthetic construct
GGAGDDNFG

SEQ ID NO: 22964 - protein, 9 aa, synthetic construct
GGEGSDSIE

SEQ ID NO: 22965 - protein, 9 aa, synthetic construct
GGVGDDAMY

SEQ ID NO: 22966 - protein, 9 aa, synthetic construct
GGVGDDAMH

SEQ ID NO: 22967 - protein, 9 aa, synthetic construct
GGAGDDNIF

SEQ ID NO: 22968 - protein, 9 aa, synthetic construct
GGVGDDALI

SEQ ID NO: 22969 - protein, 9 aa, synthetic construct
GGEGSDSIV

SEQ ID NO: 22970 - protein, 9 aa, synthetic construct
GGVGADYMN

SEQ ID NO: 22971 - protein, 9 aa, synthetic construct
GGVGADYMA

SEQ ID NO: 22972 - protein, 9 aa, synthetic construct
GGVGADYLS

SEQ ID NO: 22973 - protein, 9 aa, synthetic construct
GGVGADYID

SEQ ID NO: 22974 - protein, 9 aa, synthetic construct
GGAGDDNLK

SEQ ID NO: 22975 - protein, 9 aa, synthetic construct
GGVGADVVK

SEQ ID NO: 22976 - protein, 9 aa, synthetic construct
GGVGADVMT

SEQ ID NO: 22977 - protein, 9 aa, synthetic construct
GGVGADVMR

SEQ ID NO: 22978 - protein, 9 aa, synthetic construct
GGVGADVMN

SEQ ID NO: 22979 - protein, 9 aa, synthetic construct
GGVGADVMF

SEQ ID NO: 22980 - protein, 9 aa, synthetic construct
GGVGADVLY

SEQ ID NO: 22981 - protein, 9 aa, synthetic construct
GGVGADVLV

SEQ ID NO: 22982 - protein, 9 aa, synthetic construct
GGVGADVLH

SEQ ID NO: 22983 - protein, 9 aa, synthetic construct
GGVGADVLE

SEQ ID NO: 22984 - protein, 9 aa, synthetic construct
GGVGADVIY

SEQ ID NO: 22985 - protein, 9 aa, synthetic construct
GGVGADVID

SEQ ID NO: 22986 - protein, 9 aa, synthetic construct
GGEGSDRVI

SEQ ID NO: 22987 - protein, 9 aa, synthetic construct
GGVGDDEMY

SEQ ID NO: 22988 - protein, 9 aa, synthetic construct
GGEGSDRMF

SEQ ID NO: 22989 - protein, 9 aa, synthetic construct
GGAGDDMIF

SEQ ID NO: 22990 - protein, 9 aa, synthetic construct
GGAGDDLVT

SEQ ID NO: 22991 - protein, 9 aa, synthetic construct
GGVGDDLLS

SEQ ID NO: 22992 - protein, 9 aa, synthetic construct
GGAGDDLYM

SEQ ID NO: 22993 - protein, 9 aa, synthetic construct
GGAGDDLYS

SEQ ID NO: 22994 - protein, 9 aa, synthetic construct
GGVGDDLLG

SEQ ID NO: 22995 - protein, 9 aa, synthetic construct
GGVGDDLIV

SEQ ID NO: 22996 - protein, 9 aa, synthetic construct
GGVGDDLIE

SEQ ID NO: 22997 - protein, 9 aa, synthetic construct
GGVGDDLID

SEQ ID NO: 22998 - protein, 9 aa, synthetic construct
GGAGDDMFL

SEQ ID NO: 22999 - protein, 9 aa, synthetic construct
GGAGDDMFV

SEQ ID NO: 23000 - protein, 9 aa, synthetic construct
GGEGSDRLF

SEQ ID NO: 23001 - protein, 9 aa, synthetic construct
GGAGDDMIT

SEQ ID NO: 23002 - protein, 9 aa, synthetic construct
GGVGDDFLS

SEQ ID NO: 23003 - protein, 9 aa, synthetic construct
GGVGDDILY

SEQ ID NO: 23004 - protein, 9 aa, synthetic construct
GGAGDDMIW

SEQ ID NO: 23005 - protein, 9 aa, synthetic construct
GGVGDDILR

SEQ ID NO: 23006 - protein, 9 aa, synthetic construct
GGVGDDILQ

SEQ ID NO: 23007 - protein, 9 aa, synthetic construct
GGAGDDMLA

SEQ ID NO: 23008 - protein, 9 aa, synthetic construct
GGVGDDILF

SEQ ID NO: 23009 - protein, 9 aa, synthetic construct
GGVGDDILA

SEQ ID NO: 23010 - protein, 9 aa, synthetic construct
GGVGDDIIY

SEQ ID NO: 23011 - protein, 9 aa, synthetic construct
GGVGDDIIR

SEQ ID NO: 23012 - protein, 9 aa, synthetic construct
GGVGDDIIQ

SEQ ID NO: 23013 - protein, 9 aa, synthetic construct
GGVGDDFYR

SEQ ID NO: 23014 - protein, 9 aa, synthetic construct
GGVGEDTLS

SEQ ID NO: 23015 - protein, 9 aa, synthetic construct
GGVGEDWVA

SEQ ID NO: 23016 - protein, 9 aa, synthetic construct
GGAGDDFMG

SEQ ID NO: 23017 - protein, 9 aa, synthetic construct
GGEGSDKIA

SEQ ID NO: 23018 - protein, 9 aa, synthetic construct
GGEGSDILQ

SEQ ID NO: 23019 - protein, 9 aa, synthetic construct
GGEGSDILR

SEQ ID NO: 23020 - protein, 9 aa, synthetic construct
GGVGLDVIS

SEQ ID NO: 23021 - protein, 9 aa, synthetic construct
GGVGLDVIA

SEQ ID NO: 23022 - protein, 9 aa, synthetic construct
GGAGDDGYV

SEQ ID NO: 23023 - protein, 9 aa, synthetic construct
GGVGLDTLS

SEQ ID NO: 23024 - protein, 9 aa, synthetic construct
GGEGNDTYH

SEQ ID NO: 23025 - protein, 9 aa, synthetic construct
GGVGLDTLN

SEQ ID NO: 23026 - protein, 9 aa, synthetic construct
GGAGDDHFV

SEQ ID NO: 23027 - protein, 9 aa, synthetic construct
GGAGDDHFY

SEQ ID NO: 23028 - protein, 9 aa, synthetic construct
GGVGLDTLD

SEQ ID NO: 23029 - protein, 9 aa, synthetic construct
GGVGLDTAV

SEQ ID NO: 23030 - protein, 9 aa, synthetic construct
GGAGDDHID

SEQ ID NO: 23031 - protein, 9 aa, synthetic construct
GGAGDDHII

SEQ ID NO: 23032 - protein, 9 aa, synthetic construct
GGVGLDRLY

SEQ ID NO: 23033 - protein, 9 aa, synthetic construct
GGVGLDRLI

SEQ ID NO: 23034 - protein, 9 aa, synthetic construct
GGAGDDHIM

SEQ ID NO: 23035 - protein, 9 aa, synthetic construct
GGVGLDRAD

SEQ ID NO: 23036 - protein, 9 aa, synthetic construct
GGEGNDTVW

SEQ ID NO: 23037 - protein, 9 aa, synthetic construct
GGVGLDLIA

SEQ ID NO: 23038 - protein, 9 aa, synthetic construct
GGVGLDIVD

SEQ ID NO: 23039 - protein, 9 aa, synthetic construct
GGVGKDVLY

SEQ ID NO: 23040 - protein, 9 aa, synthetic construct
GGVGKDVID

SEQ ID NO: 23041 - protein, 9 aa, synthetic construct
GGVGKDVFF

SEQ ID NO: 23042 - protein, 9 aa, synthetic construct
GGVGKDTLG

SEQ ID NO: 23043 - protein, 9 aa, synthetic construct
GGAGDDGMI

SEQ ID NO: 23044 - protein, 9 aa, synthetic construct
GGVGMDTLT

SEQ ID NO: 23045 - protein, 9 aa, synthetic construct
GGAGDDGLL

SEQ ID NO: 23046 - protein, 9 aa, synthetic construct
GGAGDDFYI

SEQ ID NO: 23047 - protein, 9 aa, synthetic construct
GGEGNDVAK

SEQ ID NO: 23048 - protein, 9 aa, synthetic construct
GGVGNDFMS

SEQ ID NO: 23049 - protein, 9 aa, synthetic construct
GGVGNDFLS

SEQ ID NO: 23050 - protein, 9 aa, synthetic construct
GGVGNDFLL

SEQ ID NO: 23051 - protein, 9 aa, synthetic construct
GGVGNDFIS

SEQ ID NO: 23052 - protein, 9 aa, synthetic construct
GGVGNDEMQ

SEQ ID NO: 23053 - protein, 9 aa, synthetic construct
GGVGNDELW

SEQ ID NO: 23054 - protein, 9 aa, synthetic construct
GGVGNDELR

SEQ ID NO: 23055 - protein, 9 aa, synthetic construct
GGVGNDELI

SEQ ID NO: 23056 - protein, 9 aa, synthetic construct
GGAGDDFVT

SEQ ID NO: 23057 - protein, 9 aa, synthetic construct
GGVGNDEII

SEQ ID NO: 23058 - protein, 9 aa, synthetic construct
GGVGNDDLY

SEQ ID NO: 23059 - protein, 9 aa, synthetic construct
GGVGNDAIS

SEQ ID NO: 23060 - protein, 9 aa, synthetic construct
GGEGSDIIY

SEQ ID NO: 23061 - protein, 9 aa, synthetic construct
GGVGNDDLH

SEQ ID NO: 23062 - protein, 9 aa, synthetic construct
GGVGNDDLG

SEQ ID NO: 23063 - protein, 9 aa, synthetic construct
GGEGNDTYT

SEQ ID NO: 23064 - protein, 9 aa, synthetic construct
GGAGDDGFY

SEQ ID NO: 23065 - protein, 9 aa, synthetic construct
GGAGDDGID

SEQ ID NO: 23066 - protein, 9 aa, synthetic construct
GGEGSDILH

SEQ ID NO: 23067 - protein, 9 aa, synthetic construct
GGVGNDALN

SEQ ID NO: 23068 - protein, 9 aa, synthetic construct
GGAGDDGLE

SEQ ID NO: 23069 - protein, 9 aa, synthetic construct
GGVGNDALD

SEQ ID NO: 23070 - protein, 9 aa, synthetic construct
GGEGSDILK

SEQ ID NO: 23071 - protein, 9 aa, synthetic construct
GGVGKDTLF

SEQ ID NO: 23072 - protein, 9 aa, synthetic construct
GGEGSDKLR

SEQ ID NO: 23073 - protein, 9 aa, synthetic construct
GGVGEDYML

SEQ ID NO: 23074 - protein, 9 aa, synthetic construct
GGAGDDHVY

SEQ ID NO: 23075 - protein, 9 aa, synthetic construct
GGVGGDTLL

SEQ ID NO: 23076 - protein, 9 aa, synthetic construct
GGVGGDTLK

SEQ ID NO: 23077 - protein, 9 aa, synthetic construct
GGVGGDTLI

SEQ ID NO: 23078 - protein, 9 aa, synthetic construct
GGAGDDIYF

SEQ ID NO: 23079 - protein, 9 aa, synthetic construct
GGAGDDIYM

SEQ ID NO: 23080 - protein, 9 aa, synthetic construct
GGVGGDLLW

SEQ ID NO: 23081 - protein, 9 aa, synthetic construct
GGVGGDLLS

SEQ ID NO: 23082 - protein, 9 aa, synthetic construct
GGAGDDIYN

SEQ ID NO: 23083 - protein, 9 aa, synthetic construct
GGEGSDLLS

SEQ ID NO: 23084 - protein, 9 aa, synthetic construct
GGVGGDLIR

SEQ ID NO: 23085 - protein, 9 aa, synthetic construct
GGVGGDLID

SEQ ID NO: 23086 - protein, 9 aa, synthetic construct
GGVGGDILR

SEQ ID NO: 23087 - protein, 9 aa, synthetic construct
GGVGGDIFV

SEQ ID NO: 23088 - protein, 9 aa, synthetic construct
GGAGDDKFF

SEQ ID NO: 23089 - protein, 9 aa, synthetic construct
GGEGSDLLV

SEQ ID NO: 23090 - protein, 9 aa, synthetic construct
GGAGDDKFN

SEQ ID NO: 23091 - protein, 9 aa, synthetic construct
GGVGFDWLD

SEQ ID NO: 23092 - protein, 9 aa, synthetic construct
GGAGDDKIF

SEQ ID NO: 23093 - protein, 9 aa, synthetic construct
GGVGFDVFA

SEQ ID NO: 23094 - protein, 9 aa, synthetic construct
GGVGFDTMI

SEQ ID NO: 23095 - protein, 9 aa, synthetic construct
GGAGDDKII

SEQ ID NO: 23096 - protein, 9 aa, synthetic construct
GGVGFDSFD

SEQ ID NO: 23097 - protein, 9 aa, synthetic construct
GGAGDDKIN

SEQ ID NO: 23098 - protein, 9 aa, synthetic construct
GGAGDDKIV

SEQ ID NO: 23099 - protein, 9 aa, synthetic construct
GGVGFDELF

SEQ ID NO: 23100 - protein, 9 aa, synthetic construct
GGVGGDTLV

SEQ ID NO: 23101 - protein, 9 aa, synthetic construct
GGVGGDVLA

SEQ ID NO: 23102 - protein, 9 aa, synthetic construct
GGAGDDIVN

SEQ ID NO: 23103 - protein, 9 aa, synthetic construct
GGEGSDLIQ

SEQ ID NO: 23104 - protein, 9 aa, synthetic construct
GGAGDDIAD

SEQ ID NO: 23105 - protein, 9 aa, synthetic construct
GGVGKDQVT

SEQ ID NO: 23106 - protein, 9 aa, synthetic construct
GGAGDDIAI

SEQ ID NO: 23107 - protein, 9 aa, synthetic construct
GGAGDDIAN

SEQ ID NO: 23108 - protein, 9 aa, synthetic construct
GGVGKDILY

SEQ ID NO: 23109 - protein, 9 aa, synthetic construct
GGVGKDILI

SEQ ID NO: 23110 - protein, 9 aa, synthetic construct
GGVGKDIFV

SEQ ID NO: 23111 - protein, 9 aa, synthetic construct
GGVGIDTIH

SEQ ID NO: 23112 - protein, 9 aa, synthetic construct
GGVGIDTAS

SEQ ID NO: 23113 - protein, 9 aa, synthetic construct
GGVGIDTAL

SEQ ID NO: 23114 - protein, 9 aa, synthetic construct
GGVGIDTAI

SEQ ID NO: 23115 - protein, 9 aa, synthetic construct
GGVGIDTAD

SEQ ID NO: 23116 - protein, 9 aa, synthetic construct
GGAGDDIVM

SEQ ID NO: 23117 - protein, 9 aa, synthetic construct
GGAGDDIFY

SEQ ID NO: 23118 - protein, 9 aa, synthetic construct
GGAGDDIIA

SEQ ID NO: 23119 - protein, 9 aa, synthetic construct
GGAGDDIIM

SEQ ID NO: 23120 - protein, 9 aa, synthetic construct
GGVGHDTLV

SEQ ID NO: 23121 - protein, 9 aa, synthetic construct
GGVGHDTLD

SEQ ID NO: 23122 - protein, 9 aa, synthetic construct
GGEGNDTVE

SEQ ID NO: 23123 - protein, 9 aa, synthetic construct
GGAGDDIMQ

SEQ ID NO: 23124 - protein, 9 aa, synthetic construct
GGAGDDIMY

SEQ ID NO: 23125 - protein, 9 aa, synthetic construct
GGVGHDHID

SEQ ID NO: 23126 - protein, 9 aa, synthetic construct
GGVGHDELS

SEQ ID NO: 23127 - protein, 9 aa, synthetic construct
GGVGHDALY

SEQ ID NO: 23128 - protein, 9 aa, synthetic construct
GGVGVDSLH

SEQ ID NO: 23129 - protein, 9 aa, synthetic construct
GGVGVDTIN

SEQ ID NO: 23130 - protein, 9 aa, synthetic construct
GGVGVDTLA

SEQ ID NO: 23131 - protein, 9 aa, synthetic construct
GGAGADIIV

SEQ ID NO: 23132 - protein, 9 aa, synthetic construct
GGYGMDLMN

SEQ ID NO: 23133 - protein, 9 aa, synthetic construct
GGAGADHVF

SEQ ID NO: 23134 - protein, 9 aa, synthetic construct
GGYGKDVVI

SEQ ID NO: 23135 - protein, 9 aa, synthetic construct
GGAGADIAD

SEQ ID NO: 23136 - protein, 9 aa, synthetic construct
GGYGKDVLI

SEQ ID NO: 23137 - protein, 9 aa, synthetic construct
GGEGRDILV

SEQ ID NO: 23138 - protein, 9 aa, synthetic construct
GGYGKDTIN

SEQ ID NO: 23139 - protein, 9 aa, synthetic construct
GGYGKDSLN

SEQ ID NO: 23140 - protein, 9 aa, synthetic construct
GGYGKDSLF

SEQ ID NO: 23141 - protein, 9 aa, synthetic construct
GGYGKDRIQ

SEQ ID NO: 23142 - protein, 9 aa, synthetic construct
GGYGKDNLF

SEQ ID NO: 23143 - protein, 9 aa, synthetic construct
GGYGKDMIS

SEQ ID NO: 23144 - protein, 9 aa, synthetic construct
GGAGADIFE

SEQ ID NO: 23145 - protein, 9 aa, synthetic construct
GGYGKDKLY

SEQ ID NO: 23146 - protein, 9 aa, synthetic construct
GGAGADIFF

SEQ ID NO: 23147 - protein, 9 aa, synthetic construct
GGAGADIFH

SEQ ID NO: 23148 - protein, 9 aa, synthetic construct
GGYGKDFLY

SEQ ID NO: 23149 - protein, 9 aa, synthetic construct
GGAGADIFL

SEQ ID NO: 23150 - protein, 9 aa, synthetic construct
GGYGIDTVD

SEQ ID NO: 23151 - protein, 9 aa, synthetic construct
GGAGADIFN

SEQ ID NO: 23152 - protein, 9 aa, synthetic construct
GGYGIDTAD

SEQ ID NO: 23153 - protein, 9 aa, synthetic construct
GGAGADIFS

SEQ ID NO: 23154 - protein, 9 aa, synthetic construct
GGAGADIIA

SEQ ID NO: 23155 - protein, 9 aa, synthetic construct
GGYGIDLLS

SEQ ID NO: 23156 - protein, 9 aa, synthetic construct
GGAGADIIG

SEQ ID NO: 23157 - protein, 9 aa, synthetic construct
GGAGADHMD

SEQ ID NO: 23158 - protein, 9 aa, synthetic construct
GGYGNDAIV

SEQ ID NO: 23159 - protein, 9 aa, synthetic construct
GGYGNDAIY

SEQ ID NO: 23160 - protein, 9 aa, synthetic construct
GGAGADGME

SEQ ID NO: 23161 - protein, 9 aa, synthetic construct
GGAGADFVG

SEQ ID NO: 23162 - protein, 9 aa, synthetic construct
GGAGADFVN

SEQ ID NO: 23163 - protein, 9 aa, synthetic construct
GGAGADFVS

SEQ ID NO: 23164 - protein, 9 aa, synthetic construct
GGEGRDFIS

SEQ ID NO: 23165 - protein, 9 aa, synthetic construct
GGEGRDFLL

SEQ ID NO: 23166 - protein, 9 aa, synthetic construct
GGEGQDDLN

SEQ ID NO: 23167 - protein, 9 aa, synthetic construct
GGAGADGIQ

SEQ ID NO: 23168 - protein, 9 aa, synthetic construct
GGAGADGIS

SEQ ID NO: 23169 - protein, 9 aa, synthetic construct
GGAGADGLF

SEQ ID NO: 23170 - protein, 9 aa, synthetic construct
GGYGNDIYV

SEQ ID NO: 23171 - protein, 9 aa, synthetic construct
GGEGQDALS

SEQ ID NO: 23172 - protein, 9 aa, synthetic construct
GGEGRDHLS

SEQ ID NO: 23173 - protein, 9 aa, synthetic construct
GGYGNDALF

SEQ ID NO: 23174 - protein, 9 aa, synthetic construct
GGYGNDIIT

SEQ ID NO: 23175 - protein, 9 aa, synthetic construct
GGYGNDHVS

SEQ ID NO: 23176 - protein, 9 aa, synthetic construct
GGYGNDHLR

SEQ ID NO: 23177 - protein, 9 aa, synthetic construct
GGYGNDHLD

SEQ ID NO: 23178 - protein, 9 aa, synthetic construct
GGYGNDHFN

SEQ ID NO: 23179 - protein, 9 aa, synthetic construct
GGAGADHFY

SEQ ID NO: 23180 - protein, 9 aa, synthetic construct
GGYGNDEIL

SEQ ID NO: 23181 - protein, 9 aa, synthetic construct
GGYGNDEIE

SEQ ID NO: 23182 - protein, 9 aa, synthetic construct
GGAGADHLL

SEQ ID NO: 23183 - protein, 9 aa, synthetic construct
GGYGNDDLH

SEQ ID NO: 23184 - protein, 9 aa, synthetic construct
GGYGNDALR

SEQ ID NO: 23185 - protein, 9 aa, synthetic construct
GGAGADIIR

SEQ ID NO: 23186 - protein, 9 aa, synthetic construct
GGYGHDRYW

SEQ ID NO: 23187 - protein, 9 aa, synthetic construct
GGAGADFMT

SEQ ID NO: 23188 - protein, 9 aa, synthetic construct
GGYGHDRLL

SEQ ID NO: 23189 - protein, 9 aa, synthetic construct
GGYGDDTYV

SEQ ID NO: 23190 - protein, 9 aa, synthetic construct
GGYGDDTYF

SEQ ID NO: 23191 - protein, 9 aa, synthetic construct
GGYGDDTVY

SEQ ID NO: 23192 - protein, 9 aa, synthetic construct
GGYGDDTLR

SEQ ID NO: 23193 - protein, 9 aa, synthetic construct
GGYGDDTLM

SEQ ID NO: 23194 - protein, 9 aa, synthetic construct
GGYGDDTLE

SEQ ID NO: 23195 - protein, 9 aa, synthetic construct
GGYGDDTIY

SEQ ID NO: 23196 - protein, 9 aa, synthetic construct
GGAGADKLE

SEQ ID NO: 23197 - protein, 9 aa, synthetic construct
GGYGDDTIR

SEQ ID NO: 23198 - protein, 9 aa, synthetic construct
GGYGDDSVS

SEQ ID NO: 23199 - protein, 9 aa, synthetic construct
GGAGADKLR

SEQ ID NO: 23200 - protein, 9 aa, synthetic construct
GGEGPDKLI

SEQ ID NO: 23201 - protein, 9 aa, synthetic construct
GGAGADKMF

SEQ ID NO: 23202 - protein, 9 aa, synthetic construct
GGYGDDRLL

SEQ ID NO: 23203 - protein, 9 aa, synthetic construct
GGYGDDRLI

SEQ ID NO: 23204 - protein, 9 aa, synthetic construct
GGYGDDRLD

SEQ ID NO: 23205 - protein, 9 aa, synthetic construct
GGAGADKMV

SEQ ID NO: 23206 - protein, 9 aa, synthetic construct
GGEGRDLFI

SEQ ID NO: 23207 - protein, 9 aa, synthetic construct
GGYGDDQLS

SEQ ID NO: 23208 - protein, 9 aa, synthetic construct
GGAGADKYV

SEQ ID NO: 23209 - protein, 9 aa, synthetic construct
GGEGRDLIA

SEQ ID NO: 23210 - protein, 9 aa, synthetic construct
GGEGRDLIG

SEQ ID NO: 23211 - protein, 9 aa, synthetic construct
GGAGADLFH

SEQ ID NO: 23212 - protein, 9 aa, synthetic construct
GGYGDDLLR

SEQ ID NO: 23213 - protein, 9 aa, synthetic construct
GGYGDDLLH

SEQ ID NO: 23214 - protein, 9 aa, synthetic construct
GGAGADKIR

SEQ ID NO: 23215 - protein, 9 aa, synthetic construct
GGAGADKID

SEQ ID NO: 23216 - protein, 9 aa, synthetic construct
GGYGDDVIS

SEQ ID NO: 23217 - protein, 9 aa, synthetic construct
GGAGADIVI

SEQ ID NO: 23218 - protein, 9 aa, synthetic construct
GGYGHDMLD

SEQ ID NO: 23219 - protein, 9 aa, synthetic construct
GGYGHDAIT

SEQ ID NO: 23220 - protein, 9 aa, synthetic construct
GGAGADILH

SEQ ID NO: 23221 - protein, 9 aa, synthetic construct
GGYGGDVMD

SEQ ID NO: 23222 - protein, 9 aa, synthetic construct
GGYGGDHLS

SEQ ID NO: 23223 - protein, 9 aa, synthetic construct
GGEGPDTAL

SEQ ID NO: 23224 - protein, 9 aa, synthetic construct
GGYGGDELD

SEQ ID NO: 23225 - protein, 9 aa, synthetic construct
GGYGFDYLQ

SEQ ID NO: 23226 - protein, 9 aa, synthetic construct
GGYGFDTVD

SEQ ID NO: 23227 - protein, 9 aa, synthetic construct
GGYGEDVLL

SEQ ID NO: 23228 - protein, 9 aa, synthetic construct
GGYGEDVLD

SEQ ID NO: 23229 - protein, 9 aa, synthetic construct
GGAGADIVN

SEQ ID NO: 23230 - protein, 9 aa, synthetic construct
GGYGDDVIY

SEQ ID NO: 23231 - protein, 9 aa, synthetic construct
GGAGADIYT

SEQ ID NO: 23232 - protein, 9 aa, synthetic construct
GGYGDDYLS

SEQ ID NO: 23233 - protein, 9 aa, synthetic construct
GGAGADIYV

SEQ ID NO: 23234 - protein, 9 aa, synthetic construct
GGYGDDYLE

SEQ ID NO: 23235 - protein, 9 aa, synthetic construct
GGAGADKAW

SEQ ID NO: 23236 - protein, 9 aa, synthetic construct
GGAGADKFF

SEQ ID NO: 23237 - protein, 9 aa, synthetic construct
GGYGDDVVD

SEQ ID NO: 23238 - protein, 9 aa, synthetic construct
GGAGADKFH

SEQ ID NO: 23239 - protein, 9 aa, synthetic construct
GGYGDDVLR

SEQ ID NO: 23240 - protein, 9 aa, synthetic construct
GGYGDDVLL

SEQ ID NO: 23241 - protein, 9 aa, synthetic construct
GGYGDDVLE

SEQ ID NO: 23242 - protein, 9 aa, synthetic construct
GGYGNDLVL

SEQ ID NO: 23243 - protein, 9 aa, synthetic construct
GGEGRDELF

SEQ ID NO: 23244 - protein, 9 aa, synthetic construct
GGYGDDLFV

SEQ ID NO: 23245 - protein, 9 aa, synthetic construct
GGAGADEIL

SEQ ID NO: 23246 - protein, 9 aa, synthetic construct
GGAGADDID

SEQ ID NO: 23247 - protein, 9 aa, synthetic construct
GGYGSDRLG

SEQ ID NO: 23248 - protein, 9 aa, synthetic construct
GGYGSDRLE

SEQ ID NO: 23249 - protein, 9 aa, synthetic construct
GGYGSDRIN

SEQ ID NO: 23250 - protein, 9 aa, synthetic construct
GGAGADDIL

SEQ ID NO: 23251 - protein, 9 aa, synthetic construct
GGAGADDIR

SEQ ID NO: 23252 - protein, 9 aa, synthetic construct
GGYGSDLLI

SEQ ID NO: 23253 - protein, 9 aa, synthetic construct
GGYGSDILD

SEQ ID NO: 23254 - protein, 9 aa, synthetic construct
GGYGRDVLY

SEQ ID NO: 23255 - protein, 9 aa, synthetic construct
GGAGADDLQ

SEQ ID NO: 23256 - protein, 9 aa, synthetic construct
GGYGRDVLD

SEQ ID NO: 23257 - protein, 9 aa, synthetic construct
GGYGRDVIT

SEQ ID NO: 23258 - protein, 9 aa, synthetic construct
GGYGRDVIR

SEQ ID NO: 23259 - protein, 9 aa, synthetic construct
GGYGRDTLT

SEQ ID NO: 23260 - protein, 9 aa, synthetic construct
GGEGQDTLT

SEQ ID NO: 23261 - protein, 9 aa, synthetic construct
GGAGADDME

SEQ ID NO: 23262 - protein, 9 aa, synthetic construct
GGAGADDMQ

SEQ ID NO: 23263 - protein, 9 aa, synthetic construct
GGYGRDTIA

SEQ ID NO: 23264 - protein, 9 aa, synthetic construct
GGEGQDTLV

SEQ ID NO: 23265 - protein, 9 aa, synthetic construct
GGEGQDTVR

SEQ ID NO: 23266 - protein, 9 aa, synthetic construct
GGAGADEFH

SEQ ID NO: 23267 - protein, 9 aa, synthetic construct
GGEGQDVFG

SEQ ID NO: 23268 - protein, 9 aa, synthetic construct
GGAGADEFR

SEQ ID NO: 23269 - protein, 9 aa, synthetic construct
GGYGRDILV

SEQ ID NO: 23270 - protein, 9 aa, synthetic construct
GGAGADEIA

SEQ ID NO: 23271 - protein, 9 aa, synthetic construct
GGAGADDFK

SEQ ID NO: 23272 - protein, 9 aa, synthetic construct
GGYGSDSYH

SEQ ID NO: 23273 - protein, 9 aa, synthetic construct
GGYGSDTLE

SEQ ID NO: 23274 - protein, 9 aa, synthetic construct
GGYGTDRIF

SEQ ID NO: 23275 - protein, 9 aa, synthetic construct
GGYGYDTID

SEQ ID NO: 23276 - protein, 9 aa, synthetic construct
GGEGQDRLE

SEQ ID NO: 23277 - protein, 9 aa, synthetic construct
GGAGADAFL

SEQ ID NO: 23278 - protein, 9 aa, synthetic construct
GGYGWDSLE

SEQ ID NO: 23279 - protein, 9 aa, synthetic construct
GGYGWDEIH

SEQ ID NO: 23280 - protein, 9 aa, synthetic construct
GGAGADAIA

SEQ ID NO: 23281 - protein, 9 aa, synthetic construct
GGYGVDVLN

SEQ ID NO: 23282 - protein, 9 aa, synthetic construct
GGAGADAIN

SEQ ID NO: 23283 - protein, 9 aa, synthetic construct
GGYGTDTIW

SEQ ID NO: 23284 - protein, 9 aa, synthetic construct
GGAGADALQ

SEQ ID NO: 23285 - protein, 9 aa, synthetic construct
GGYGTDSMF

SEQ ID NO: 23286 - protein, 9 aa, synthetic construct
GGYGTDILN

SEQ ID NO: 23287 - protein, 9 aa, synthetic construct
GGAGADAVS

SEQ ID NO: 23288 - protein, 9 aa, synthetic construct
GGAGADAMG

SEQ ID NO: 23289 - protein, 9 aa, synthetic construct
GGYGSDYLS

SEQ ID NO: 23290 - protein, 9 aa, synthetic construct
GGAGADAMH

SEQ ID NO: 23291 - protein, 9 aa, synthetic construct
GGYGSDVLN

SEQ ID NO: 23292 - protein, 9 aa, synthetic construct
GGYGSDVLL

SEQ ID NO: 23293 - protein, 9 aa, synthetic construct
GGAGADAML

SEQ ID NO: 23294 - protein, 9 aa, synthetic construct
GGYGSDTVL

SEQ ID NO: 23295 - protein, 9 aa, synthetic construct
GGEGQDSLY

SEQ ID NO: 23296 - protein, 9 aa, synthetic construct
GGYGSDTLW

SEQ ID NO: 23297 - protein, 9 aa, synthetic construct
GGYGSDTLT

SEQ ID NO: 23298 - protein, 9 aa, synthetic construct
GGYGSDTLR

SEQ ID NO: 23299 - protein, 9 aa, synthetic construct
GGEGQDVLF

SEQ ID NO: 23300 - protein, 9 aa, synthetic construct
GGEGQDVLL

SEQ ID NO: 23301 - protein, 9 aa, synthetic construct
GGYGNDMVS

SEQ ID NO: 23302 - protein, 9 aa, synthetic construct
GGAGADEIR

SEQ ID NO: 23303 - protein, 9 aa, synthetic construct
GGYGNDTIQ

SEQ ID NO: 23304 - protein, 9 aa, synthetic construct
GGYGNDTIL

SEQ ID NO: 23305 - protein, 9 aa, synthetic construct
GGEGRDALI

SEQ ID NO: 23306 - protein, 9 aa, synthetic construct
GGYGNDSYY

SEQ ID NO: 23307 - protein, 9 aa, synthetic construct
GGEGRDAVF

SEQ ID NO: 23308 - protein, 9 aa, synthetic construct
GGYGNDSMT

SEQ ID NO: 23309 - protein, 9 aa, synthetic construct
GGEGQDILF

SEQ ID NO: 23310 - protein, 9 aa, synthetic construct
GGAGADFFV

SEQ ID NO: 23311 - protein, 9 aa, synthetic construct
GGAGADFIA

SEQ ID NO: 23312 - protein, 9 aa, synthetic construct
GGYGNDRVN

SEQ ID NO: 23313 - protein, 9 aa, synthetic construct
GGYGNDRLR

SEQ ID NO: 23314 - protein, 9 aa, synthetic construct
GGAGADFIY

SEQ ID NO: 23315 - protein, 9 aa, synthetic construct
GGAGADFLF

SEQ ID NO: 23316 - protein, 9 aa, synthetic construct
GGEGQDHLM

SEQ ID NO: 23317 - protein, 9 aa, synthetic construct
GGYGNDRIA

SEQ ID NO: 23318 - protein, 9 aa, synthetic construct
GGEGRDDLR

SEQ ID NO: 23319 - protein, 9 aa, synthetic construct
GGYGNDQVS

SEQ ID NO: 23320 - protein, 9 aa, synthetic construct
GGAGADFLI

SEQ ID NO: 23321 - protein, 9 aa, synthetic construct
GGYGNDQLY

SEQ ID NO: 23322 - protein, 9 aa, synthetic construct
GGEGRDDML

SEQ ID NO: 23323 - protein, 9 aa, synthetic construct
GGYGNDQLR

SEQ ID NO: 23324 - protein, 9 aa, synthetic construct
GGYGNDQLN

SEQ ID NO: 23325 - protein, 9 aa, synthetic construct
GGAGADFLN

SEQ ID NO: 23326 - protein, 9 aa, synthetic construct
GGAGADFLW

SEQ ID NO: 23327 - protein, 9 aa, synthetic construct
GGAGADFMD

SEQ ID NO: 23328 - protein, 9 aa, synthetic construct
GGEGRDAFV

SEQ ID NO: 23329 - protein, 9 aa, synthetic construct
GGEGQDKLY

SEQ ID NO: 23330 - protein, 9 aa, synthetic construct
GGYGNDTLG

SEQ ID NO: 23331 - protein, 9 aa, synthetic construct
GGAGADEMA

SEQ ID NO: 23332 - protein, 9 aa, synthetic construct
GGYGQDTIN

SEQ ID NO: 23333 - protein, 9 aa, synthetic construct
GGAGADELG

SEQ ID NO: 23334 - protein, 9 aa, synthetic construct
GGEGQDVLS

SEQ ID NO: 23335 - protein, 9 aa, synthetic construct
GGYGQDLID

SEQ ID NO: 23336 - protein, 9 aa, synthetic construct
GGEGQDVLY

SEQ ID NO: 23337 - protein, 9 aa, synthetic construct
GGYGQDFLD

SEQ ID NO: 23338 - protein, 9 aa, synthetic construct
GGYGQDELW

SEQ ID NO: 23339 - protein, 9 aa, synthetic construct
GGYGPDTFV

SEQ ID NO: 23340 - protein, 9 aa, synthetic construct
GGAGADELM

SEQ ID NO: 23341 - protein, 9 aa, synthetic construct
GGYGNDWME

SEQ ID NO: 23342 - protein, 9 aa, synthetic construct
GGYGNDWLD

SEQ ID NO: 23343 - protein, 9 aa, synthetic construct
GGYGNDVMT

SEQ ID NO: 23344 - protein, 9 aa, synthetic construct
GGEGQDYLV

SEQ ID NO: 23345 - protein, 9 aa, synthetic construct
GGYGNDVMA

SEQ ID NO: 23346 - protein, 9 aa, synthetic construct
GGYGNDVLY

SEQ ID NO: 23347 - protein, 9 aa, synthetic construct
GGAGADEMH

SEQ ID NO: 23348 - protein, 9 aa, synthetic construct
GGYGNDVLL

SEQ ID NO: 23349 - protein, 9 aa, synthetic construct
GGAGADEMI

SEQ ID NO: 23350 - protein, 9 aa, synthetic construct
GGAGADEMR

SEQ ID NO: 23351 - protein, 9 aa, synthetic construct
GGAGADEMT

SEQ ID NO: 23352 - protein, 9 aa, synthetic construct
GGYGNDTYH

SEQ ID NO: 23353 - protein, 9 aa, synthetic construct
GGAGADEMW

SEQ ID NO: 23354 - protein, 9 aa, synthetic construct
GGYGNDTVQ

SEQ ID NO: 23355 - protein, 9 aa, synthetic construct
GGYGNDTVM

SEQ ID NO: 23356 - protein, 9 aa, synthetic construct
GGYGDDLIH

SEQ ID NO: 23357 - protein, 9 aa, synthetic construct
GGAGADLIM

SEQ ID NO: 23358 - protein, 9 aa, synthetic construct
GGVGVDTLI

SEQ ID NO: 23359 - protein, 9 aa, synthetic construct
GGWGDDVLE

SEQ ID NO: 23360 - protein, 9 aa, synthetic construct
GGWGKDELT

SEQ ID NO: 23361 - protein, 9 aa, synthetic construct
GGAGADSFH

SEQ ID NO: 23362 - protein, 9 aa, synthetic construct
GGEGNDWLS

SEQ ID NO: 23363 - protein, 9 aa, synthetic construct
GGAGADSFT

SEQ ID NO: 23364 - protein, 9 aa, synthetic construct
GGWGHDTLV

SEQ ID NO: 23365 - protein, 9 aa, synthetic construct
GGWGHDQLA

SEQ ID NO: 23366 - protein, 9 aa, synthetic construct
GGWGHDLVN

SEQ ID NO: 23367 - protein, 9 aa, synthetic construct
GGAGADSIM

SEQ ID NO: 23368 - protein, 9 aa, synthetic construct
GGWGGDVLK

SEQ ID NO: 23369 - protein, 9 aa, synthetic construct
GGWGGDTLE

SEQ ID NO: 23370 - protein, 9 aa, synthetic construct
GGAGADSIV

SEQ ID NO: 23371 - protein, 9 aa, synthetic construct
GGWGEDYLD

SEQ ID NO: 23372 - protein, 9 aa, synthetic construct
GGWGEDLLK

SEQ ID NO: 23373 - protein, 9 aa, synthetic construct
GGWGEDLLE

SEQ ID NO: 23374 - protein, 9 aa, synthetic construct
GGWGEDIVD

SEQ ID NO: 23375 - protein, 9 aa, synthetic construct
GGAGADSLW

SEQ ID NO: 23376 - protein, 9 aa, synthetic construct
GGWGDDYFH

SEQ ID NO: 23377 - protein, 9 aa, synthetic construct
GGWGDDWLG

SEQ ID NO: 23378 - protein, 9 aa, synthetic construct
GGWGDDWLA

SEQ ID NO: 23379 - protein, 9 aa, synthetic construct
GGAGADSMN

SEQ ID NO: 23380 - protein, 9 aa, synthetic construct
GGWGDDVVV

SEQ ID NO: 23381 - protein, 9 aa, synthetic construct
GGWGDDVVN

SEQ ID NO: 23382 - protein, 9 aa, synthetic construct
GGWGDDVMT

SEQ ID NO: 23383 - protein, 9 aa, synthetic construct
GGAGADSMW

SEQ ID NO: 23384 - protein, 9 aa, synthetic construct
GGAGADSMY

SEQ ID NO: 23385 - protein, 9 aa, synthetic construct
GGAGADSFA

SEQ ID NO: 23386 - protein, 9 aa, synthetic construct
GGAGADSAT

SEQ ID NO: 23387 - protein, 9 aa, synthetic construct
GGWGKDLLV

SEQ ID NO: 23388 - protein, 9 aa, synthetic construct
GGWGNDLLE

SEQ ID NO: 23389 - protein, 9 aa, synthetic construct
GGWGNDRLS

SEQ ID NO: 23390 - protein, 9 aa, synthetic construct
GGWGNDRLD

SEQ ID NO: 23391 - protein, 9 aa, synthetic construct
GGWGNDRIL

SEQ ID NO: 23392 - protein, 9 aa, synthetic construct
GGAGADRIS

SEQ ID NO: 23393 - protein, 9 aa, synthetic construct
GGWGNDQLI

SEQ ID NO: 23394 - protein, 9 aa, synthetic construct
GGAGADRIV

SEQ ID NO: 23395 - protein, 9 aa, synthetic construct
GGWGNDMLA

SEQ ID NO: 23396 - protein, 9 aa, synthetic construct
GGWGNDLYL

SEQ ID NO: 23397 - protein, 9 aa, synthetic construct
GGWGNDLLV

SEQ ID NO: 23398 - protein, 9 aa, synthetic construct
GGWGNDLLN

SEQ ID NO: 23399 - protein, 9 aa, synthetic construct
GGWGNDLLI

SEQ ID NO: 23400 - protein, 9 aa, synthetic construct
GGWGNDKLD

SEQ ID NO: 23401 - protein, 9 aa, synthetic construct
GGWGKDMLA

SEQ ID NO: 23402 - protein, 9 aa, synthetic construct
GGWGNDIIH

SEQ ID NO: 23403 - protein, 9 aa, synthetic construct
GGWGNDIID

SEQ ID NO: 23404 - protein, 9 aa, synthetic construct
GGWGNDELL

SEQ ID NO: 23405 - protein, 9 aa, synthetic construct
GGEGRDSLD

SEQ ID NO: 23406 - protein, 9 aa, synthetic construct
GGWGMDVLY

SEQ ID NO: 23407 - protein, 9 aa, synthetic construct
GGWGMDTMT

SEQ ID NO: 23408 - protein, 9 aa, synthetic construct
GGWGLDVVS

SEQ ID NO: 23409 - protein, 9 aa, synthetic construct
GGAGADRMW

SEQ ID NO: 23410 - protein, 9 aa, synthetic construct
GGEGRDSLE

SEQ ID NO: 23411 - protein, 9 aa, synthetic construct
GGAGADRVH

SEQ ID NO: 23412 - protein, 9 aa, synthetic construct
GGEGRDSLV

SEQ ID NO: 23413 - protein, 9 aa, synthetic construct
GGAGADSVD

SEQ ID NO: 23414 - protein, 9 aa, synthetic construct
GGWGDDVIN

SEQ ID NO: 23415 - protein, 9 aa, synthetic construct
GGWGNDSLS

SEQ ID NO: 23416 - protein, 9 aa, synthetic construct
GGWGDDVIL

SEQ ID NO: 23417 - protein, 9 aa, synthetic construct
GGWGADVFV

SEQ ID NO: 23418 - protein, 9 aa, synthetic construct
GGWGADTLD

SEQ ID NO: 23419 - protein, 9 aa, synthetic construct
GGWGADTIE

SEQ ID NO: 23420 - protein, 9 aa, synthetic construct
GGAGADTMH

SEQ ID NO: 23421 - protein, 9 aa, synthetic construct
GGEGRDTIL

SEQ ID NO: 23422 - protein, 9 aa, synthetic construct
GGWGADRLS

SEQ ID NO: 23423 - protein, 9 aa, synthetic construct
GGWGADQLT

SEQ ID NO: 23424 - protein, 9 aa, synthetic construct
GGWGADLLT

SEQ ID NO: 23425 - protein, 9 aa, synthetic construct
GGWGADLLR

SEQ ID NO: 23426 - protein, 9 aa, synthetic construct
GGEGRDTIN

SEQ ID NO: 23427 - protein, 9 aa, synthetic construct
GGAGADTVM

SEQ ID NO: 23428 - protein, 9 aa, synthetic construct
GGWGADAIR

SEQ ID NO: 23429 - protein, 9 aa, synthetic construct
GGWGADAFV

SEQ ID NO: 23430 - protein, 9 aa, synthetic construct
GGAGADTVV

SEQ ID NO: 23431 - protein, 9 aa, synthetic construct
GGEGRDTIS

SEQ ID NO: 23432 - protein, 9 aa, synthetic construct
GGVGYDSLY

SEQ ID NO: 23433 - protein, 9 aa, synthetic construct
GGVGYDSLS

SEQ ID NO: 23434 - protein, 9 aa, synthetic construct
GGEGRDTIY

SEQ ID NO: 23435 - protein, 9 aa, synthetic construct
GGVGYDRLR

SEQ ID NO: 23436 - protein, 9 aa, synthetic construct
GGVGYDLLD

SEQ ID NO: 23437 - protein, 9 aa, synthetic construct
GGAGADTYL

SEQ ID NO: 23438 - protein, 9 aa, synthetic construct
GGAGADTYT

SEQ ID NO: 23439 - protein, 9 aa, synthetic construct
GGVGVDWVT

SEQ ID NO: 23440 - protein, 9 aa, synthetic construct
GGVGVDTLT

SEQ ID NO: 23441 - protein, 9 aa, synthetic construct
GGEGRDTLE

SEQ ID NO: 23442 - protein, 9 aa, synthetic construct
GGWGADVLH

SEQ ID NO: 23443 - protein, 9 aa, synthetic construct
GGWGADVLN

SEQ ID NO: 23444 - protein, 9 aa, synthetic construct
GGWGADVLR

SEQ ID NO: 23445 - protein, 9 aa, synthetic construct
GGWGDDSLS

SEQ ID NO: 23446 - protein, 9 aa, synthetic construct
GGAGADSVM

SEQ ID NO: 23447 - protein, 9 aa, synthetic construct
GGWGDDTYI

SEQ ID NO: 23448 - protein, 9 aa, synthetic construct
GGEGRDTFF

SEQ ID NO: 23449 - protein, 9 aa, synthetic construct
GGWGDDTLT

SEQ ID NO: 23450 - protein, 9 aa, synthetic construct
GGAGADTAL

SEQ ID NO: 23451 - protein, 9 aa, synthetic construct
GGWGDDTLN

SEQ ID NO: 23452 - protein, 9 aa, synthetic construct
GGWGDDTLK

SEQ ID NO: 23453 - protein, 9 aa, synthetic construct
GGWGDDTLI

SEQ ID NO: 23454 - protein, 9 aa, synthetic construct
GGWGDDTLA

SEQ ID NO: 23455 - protein, 9 aa, synthetic construct
GGWGDDTFV

SEQ ID NO: 23456 - protein, 9 aa, synthetic construct
GGWGDDSMH

SEQ ID NO: 23457 - protein, 9 aa, synthetic construct
GGWGDDSLD

SEQ ID NO: 23458 - protein, 9 aa, synthetic construct
GGWGDDAIT

SEQ ID NO: 23459 - protein, 9 aa, synthetic construct
GGWGDDSIL

SEQ ID NO: 23460 - protein, 9 aa, synthetic construct
GGWGDDRME

SEQ ID NO: 23461 - protein, 9 aa, synthetic construct
GGWGDDRLT

SEQ ID NO: 23462 - protein, 9 aa, synthetic construct
GGWGDDRIE

SEQ ID NO: 23463 - protein, 9 aa, synthetic construct
GGWGDDLVY

SEQ ID NO: 23464 - protein, 9 aa, synthetic construct
GGWGDDLVS

SEQ ID NO: 23465 - protein, 9 aa, synthetic construct
GGWGDDIVY

SEQ ID NO: 23466 - protein, 9 aa, synthetic construct
GGAGADTIQ

SEQ ID NO: 23467 - protein, 9 aa, synthetic construct
GGEGNDVYW

SEQ ID NO: 23468 - protein, 9 aa, synthetic construct
GGWGDDELL

SEQ ID NO: 23469 - protein, 9 aa, synthetic construct
GGWGDDALS

SEQ ID NO: 23470 - protein, 9 aa, synthetic construct
GGWGNDSIY

SEQ ID NO: 23471 - protein, 9 aa, synthetic construct
GGWGNDSLY

SEQ ID NO: 23472 - protein, 9 aa, synthetic construct
GGEGRDLLI

SEQ ID NO: 23473 - protein, 9 aa, synthetic construct
GGXGNDYLE

SEQ ID NO: 23474 - protein, 9 aa, synthetic construct
GGAGADMAS

SEQ ID NO: 23475 - protein, 9 aa, synthetic construct
GGYGADTIL

SEQ ID NO: 23476 - protein, 9 aa, synthetic construct
GGYGADSLT

SEQ ID NO: 23477 - protein, 9 aa, synthetic construct
GGAGADMIL

SEQ ID NO: 23478 - protein, 9 aa, synthetic construct
GGYGADRMV

SEQ ID NO: 23479 - protein, 9 aa, synthetic construct
GGYGADRLY

SEQ ID NO: 23480 - protein, 9 aa, synthetic construct
GGEGNDYLW

SEQ ID NO: 23481 - protein, 9 aa, synthetic construct
GGYGADRLQ

SEQ ID NO: 23482 - protein, 9 aa, synthetic construct
GGYGADRLA

SEQ ID NO: 23483 - protein, 9 aa, synthetic construct
GGYGADQMS

SEQ ID NO: 23484 - protein, 9 aa, synthetic construct
GGAGADMLE

SEQ ID NO: 23485 - protein, 9 aa, synthetic construct
GGYGADLLR

SEQ ID NO: 23486 - protein, 9 aa, synthetic construct
GGAGADMLR

SEQ ID NO: 23487 - protein, 9 aa, synthetic construct
GGYGADLLF

SEQ ID NO: 23488 - protein, 9 aa, synthetic construct
GGYGADLLD

SEQ ID NO: 23489 - protein, 9 aa, synthetic construct
GGYGADLLA

SEQ ID NO: 23490 - protein, 9 aa, synthetic construct
GGYGADLIY

SEQ ID NO: 23491 - protein, 9 aa, synthetic construct
GGEGNDYLR

SEQ ID NO: 23492 - protein, 9 aa, synthetic construct
GGAGADMMT

SEQ ID NO: 23493 - protein, 9 aa, synthetic construct
GGEGNDYLQ

SEQ ID NO: 23494 - protein, 9 aa, synthetic construct
GGYGADIID

SEQ ID NO: 23495 - protein, 9 aa, synthetic construct
GGEGRDQFS

SEQ ID NO: 23496 - protein, 9 aa, synthetic construct
GGEGNDYLL

SEQ ID NO: 23497 - protein, 9 aa, synthetic construct
GGAGADNIN

SEQ ID NO: 23498 - protein, 9 aa, synthetic construct
GGEGRDQIN

SEQ ID NO: 23499 - protein, 9 aa, synthetic construct
GGEGRDLMI

SEQ ID NO: 23500 - protein, 9 aa, synthetic construct
GGYGADTLH

SEQ ID NO: 23501 - protein, 9 aa, synthetic construct
GGAGADLYF

SEQ ID NO: 23502 - protein, 9 aa, synthetic construct
GGAGADLMF

SEQ ID NO: 23503 - protein, 9 aa, synthetic construct
GGYGDDIYY

SEQ ID NO: 23504 - protein, 9 aa, synthetic construct
GGYGDDILV

SEQ ID NO: 23505 - protein, 9 aa, synthetic construct
GGAGADLIT

SEQ ID NO: 23506 - protein, 9 aa, synthetic construct
GGYGDDHLL

SEQ ID NO: 23507 - protein, 9 aa, synthetic construct
GGYGDDFLT

SEQ ID NO: 23508 - protein, 9 aa, synthetic construct
GGAGADLLM

SEQ ID NO: 23509 - protein, 9 aa, synthetic construct
GGYGDDELH

SEQ ID NO: 23510 - protein, 9 aa, synthetic construct
GGYGDDEIN

SEQ ID NO: 23511 - protein, 9 aa, synthetic construct
GGEGRDLLM

SEQ ID NO: 23512 - protein, 9 aa, synthetic construct
GGYGDDAVS

SEQ ID NO: 23513 - protein, 9 aa, synthetic construct
GGYGDDALY

SEQ ID NO: 23514 - protein, 9 aa, synthetic construct
GGEGNDYVD

SEQ ID NO: 23515 - protein, 9 aa, synthetic construct
GGYGADTLV

SEQ ID NO: 23516 - protein, 9 aa, synthetic construct
GGYGADWLD

SEQ ID NO: 23517 - protein, 9 aa, synthetic construct
GGYGADVLS

SEQ ID NO: 23518 - protein, 9 aa, synthetic construct
GGYGADVLR

SEQ ID NO: 23519 - protein, 9 aa, synthetic construct
GGYGADVLK

SEQ ID NO: 23520 - protein, 9 aa, synthetic construct
GGYGADVID

SEQ ID NO: 23521 - protein, 9 aa, synthetic construct
GGYGADVFV

SEQ ID NO: 23522 - protein, 9 aa, synthetic construct
GGYGADTYV

SEQ ID NO: 23523 - protein, 9 aa, synthetic construct
GGEGRDLLY

SEQ ID NO: 23524 - protein, 9 aa, synthetic construct
GGYGADTVT

SEQ ID NO: 23525 - protein, 9 aa, synthetic construct
GGAGADLVL

SEQ ID NO: 23526 - protein, 9 aa, synthetic construct
GGAGADLVS

SEQ ID NO: 23527 - protein, 9 aa, synthetic construct
GGXGSDTLR

SEQ ID NO: 23528 - protein, 9 aa, synthetic construct
GGXGNDLLF

SEQ ID NO: 23529 - protein, 9 aa, synthetic construct
GGWGNDTIA

SEQ ID NO: 23530 - protein, 9 aa, synthetic construct
GGEGRDQLI

SEQ ID NO: 23531 - protein, 9 aa, synthetic construct
GGWGRDTLS

SEQ ID NO: 23532 - protein, 9 aa, synthetic construct
GGWGRDTIT

SEQ ID NO: 23533 - protein, 9 aa, synthetic construct
GGWGRDTIN

SEQ ID NO: 23534 - protein, 9 aa, synthetic construct
GGWGRDTIK

SEQ ID NO: 23535 - protein, 9 aa, synthetic construct
GGWGRDTIH

SEQ ID NO: 23536 - protein, 9 aa, synthetic construct
GGWGRDRLY

SEQ ID NO: 23537 - protein, 9 aa, synthetic construct
GGWGRDLIL

SEQ ID NO: 23538 - protein, 9 aa, synthetic construct
GGAGADQMH

SEQ ID NO: 23539 - protein, 9 aa, synthetic construct
GGWGQDTVA

SEQ ID NO: 23540 - protein, 9 aa, synthetic construct
GGAGADQML

SEQ ID NO: 23541 - protein, 9 aa, synthetic construct
GGWGQDLMT

SEQ ID NO: 23542 - protein, 9 aa, synthetic construct
GGEGRDRLS

SEQ ID NO: 23543 - protein, 9 aa, synthetic construct
GGEGRDRME

SEQ ID NO: 23544 - protein, 9 aa, synthetic construct
GGEGNDYIE

SEQ ID NO: 23545 - protein, 9 aa, synthetic construct
GGWGNDVVI

SEQ ID NO: 23546 - protein, 9 aa, synthetic construct
GGWGNDVLS

SEQ ID NO: 23547 - protein, 9 aa, synthetic construct
GGEGRDRVD

SEQ ID NO: 23548 - protein, 9 aa, synthetic construct
GGAGADRAW

SEQ ID NO: 23549 - protein, 9 aa, synthetic construct
GGWGNDVFE

SEQ ID NO: 23550 - protein, 9 aa, synthetic construct
GGWGNDTVE

SEQ ID NO: 23551 - protein, 9 aa, synthetic construct
GGWGNDTVD

SEQ ID NO: 23552 - protein, 9 aa, synthetic construct
GGWGNDTMN

SEQ ID NO: 23553 - protein, 9 aa, synthetic construct
GGWGNDTLK

SEQ ID NO: 23554 - protein, 9 aa, synthetic construct
GGWGNDTIN

SEQ ID NO: 23555 - protein, 9 aa, synthetic construct
GGAGADRFR

SEQ ID NO: 23556 - protein, 9 aa, synthetic construct
GGWGRDTVA

SEQ ID NO: 23557 - protein, 9 aa, synthetic construct
GGAGADQLK

SEQ ID NO: 23558 - protein, 9 aa, synthetic construct
GGAGADQLH

SEQ ID NO: 23559 - protein, 9 aa, synthetic construct
GGAGADQFH

SEQ ID NO: 23560 - protein, 9 aa, synthetic construct
GGXGADXID

SEQ ID NO: 23561 - protein, 9 aa, synthetic construct
GGXGADILI

SEQ ID NO: 23562 - protein, 9 aa, synthetic construct
GGAGADNLW

SEQ ID NO: 23563 - protein, 9 aa, synthetic construct
GGAGADNMD

SEQ ID NO: 23564 - protein, 9 aa, synthetic construct
GGWGYDDLI

SEQ ID NO: 23565 - protein, 9 aa, synthetic construct
GGWGWDELI

SEQ ID NO: 23566 - protein, 9 aa, synthetic construct
GGWGVDVLR

SEQ ID NO: 23567 - protein, 9 aa, synthetic construct
GGWGVDTMR

SEQ ID NO: 23568 - protein, 9 aa, synthetic construct
GGAGADNVN

SEQ ID NO: 23569 - protein, 9 aa, synthetic construct
GGAGADQAS

SEQ ID NO: 23570 - protein, 9 aa, synthetic construct
GGAGADQAT

SEQ ID NO: 23571 - protein, 9 aa, synthetic construct
GGEGNDYIY

SEQ ID NO: 23572 - protein, 9 aa, synthetic construct
GGWGSDCFV

SEQ ID NO: 23573 - protein, 9 aa, synthetic construct
GGWGSDTLY

SEQ ID NO: 23574 - protein, 9 aa, synthetic construct
GGWGSDTLR

SEQ ID NO: 23575 - protein, 9 aa, synthetic construct
GGWGSDTLD

SEQ ID NO: 23576 - protein, 9 aa, synthetic construct
GGAGADQIA

SEQ ID NO: 23577 - protein, 9 aa, synthetic construct
GGWGSDSLS

SEQ ID NO: 23578 - protein, 9 aa, synthetic construct
GGEGRDRIW

SEQ ID NO: 23579 - protein, 9 aa, synthetic construct
GGAGADQIH

SEQ ID NO: 23580 - protein, 9 aa, synthetic construct
GGAGADQII

SEQ ID NO: 23581 - protein, 9 aa, synthetic construct
GGAGADQIT

SEQ ID NO: 23582 - protein, 9 aa, synthetic construct
GGWGSDLIY

SEQ ID NO: 23583 - protein, 9 aa, synthetic construct
GGWGSDILV

SEQ ID NO: 23584 - protein, 9 aa, synthetic construct
GGAGDDNVG

SEQ ID NO: 23585 - protein, 9 aa, synthetic construct
GGAGDDNYV

SEQ ID NO: 23586 - protein, 9 aa, synthetic construct
GGFGADILI

SEQ ID NO: 23587 - protein, 9 aa, synthetic construct
GGEGNDRFD

SEQ ID NO: 23588 - protein, 9 aa, synthetic construct
GGTGNDIVR

SEQ ID NO: 23589 - protein, 9 aa, synthetic construct
GGTGNDIVF

SEQ ID NO: 23590 - protein, 9 aa, synthetic construct
GGTGNDIVD

SEQ ID NO: 23591 - protein, 9 aa, synthetic construct
GGEGVDLLL

SEQ ID NO: 23592 - protein, 9 aa, synthetic construct
GGTGNDIMS

SEQ ID NO: 23593 - protein, 9 aa, synthetic construct
GGTGNDIMI

SEQ ID NO: 23594 - protein, 9 aa, synthetic construct
GGEGVDLLQ

SEQ ID NO: 23595 - protein, 9 aa, synthetic construct
GGTGNDILM

SEQ ID NO: 23596 - protein, 9 aa, synthetic construct
GGTGNDIIV

SEQ ID NO: 23597 - protein, 9 aa, synthetic construct
GGTGNDIII

SEQ ID NO: 23598 - protein, 9 aa, synthetic construct
GGTGNDIIG

SEQ ID NO: 23599 - protein, 9 aa, synthetic construct
GGTGNDIFR

SEQ ID NO: 23600 - protein, 9 aa, synthetic construct
GGTGNDIFQ

SEQ ID NO: 23601 - protein, 9 aa, synthetic construct
GGAGFDLIQ

SEQ ID NO: 23602 - protein, 9 aa, synthetic construct
GGAGFDLLI

SEQ ID NO: 23603 - protein, 9 aa, synthetic construct
GGAGFDLLL

SEQ ID NO: 23604 - protein, 9 aa, synthetic construct
GGAGFDLLT

SEQ ID NO: 23605 - protein, 9 aa, synthetic construct
GGTGNDHME

SEQ ID NO: 23606 - protein, 9 aa, synthetic construct
GGAGFDLMY

SEQ ID NO: 23607 - protein, 9 aa, synthetic construct
GGAGFDLVI

SEQ ID NO: 23608 - protein, 9 aa, synthetic construct
GGAGFDMAS

SEQ ID NO: 23609 - protein, 9 aa, synthetic construct
GGAGFDMIY

SEQ ID NO: 23610 - protein, 9 aa, synthetic construct
GGAGFDMLY

SEQ ID NO: 23611 - protein, 9 aa, synthetic construct
GGAGFDMVD

SEQ ID NO: 23612 - protein, 9 aa, synthetic construct
GGEGVDRAV

SEQ ID NO: 23613 - protein, 9 aa, synthetic construct
GGTGNDIVY

SEQ ID NO: 23614 - protein, 9 aa, synthetic construct
GGTGNDIYN

SEQ ID NO: 23615 - protein, 9 aa, synthetic construct
GGVGADTVS

SEQ ID NO: 23616 - protein, 9 aa, synthetic construct
GGAGFDIYK

SEQ ID NO: 23617 - protein, 9 aa, synthetic construct
GGTGNDLML

SEQ ID NO: 23618 - protein, 9 aa, synthetic construct
GGEGVDIVL

SEQ ID NO: 23619 - protein, 9 aa, synthetic construct
GGTGNDLMD

SEQ ID NO: 23620 - protein, 9 aa, synthetic construct
GGTGNDLLW

SEQ ID NO: 23621 - protein, 9 aa, synthetic construct
GGTGNDLIV

SEQ ID NO: 23622 - protein, 9 aa, synthetic construct
GGEGNDRFV

SEQ ID NO: 23623 - protein, 9 aa, synthetic construct
GGTGNDLIR

SEQ ID NO: 23624 - protein, 9 aa, synthetic construct
GGTGNDLIL

SEQ ID NO: 23625 - protein, 9 aa, synthetic construct
GGTGNDLII

SEQ ID NO: 23626 - protein, 9 aa, synthetic construct
GGTGNDLIG

SEQ ID NO: 23627 - protein, 9 aa, synthetic construct
GGAGFDIIQ

SEQ ID NO: 23628 - protein, 9 aa, synthetic construct
GGTGNDLAF

SEQ ID NO: 23629 - protein, 9 aa, synthetic construct
GGTGNDLAD

SEQ ID NO: 23630 - protein, 9 aa, synthetic construct
GGTGNDKYY

SEQ ID NO: 23631 - protein, 9 aa, synthetic construct
GGEGVDLLA

SEQ ID NO: 23632 - protein, 9 aa, synthetic construct
GGTGNDKVL

SEQ ID NO: 23633 - protein, 9 aa, synthetic construct
GGTGNDKLW

SEQ ID NO: 23634 - protein, 9 aa, synthetic construct
GGTGNDKLQ

SEQ ID NO: 23635 - protein, 9 aa, synthetic construct
GGTGNDKLK

SEQ ID NO: 23636 - protein, 9 aa, synthetic construct
GGTGNDKLH

SEQ ID NO: 23637 - protein, 9 aa, synthetic construct
GGAGFDILT

SEQ ID NO: 23638 - protein, 9 aa, synthetic construct
GGAGFDILV

SEQ ID NO: 23639 - protein, 9 aa, synthetic construct
GGAGFDILY

SEQ ID NO: 23640 - protein, 9 aa, synthetic construct
GGTGNDKIN

SEQ ID NO: 23641 - protein, 9 aa, synthetic construct
GGAGFDIVS

SEQ ID NO: 23642 - protein, 9 aa, synthetic construct
GGAGFDNFV

SEQ ID NO: 23643 - protein, 9 aa, synthetic construct
GGTGNDFVG

SEQ ID NO: 23644 - protein, 9 aa, synthetic construct
GGAGFDNLY

SEQ ID NO: 23645 - protein, 9 aa, synthetic construct
GGAGFDQLF

SEQ ID NO: 23646 - protein, 9 aa, synthetic construct
GGTGNDDLH

SEQ ID NO: 23647 - protein, 9 aa, synthetic construct
GGTGNDDLE

SEQ ID NO: 23648 - protein, 9 aa, synthetic construct
GGAGFDSLD

SEQ ID NO: 23649 - protein, 9 aa, synthetic construct
GGTGNDDIT

SEQ ID NO: 23650 - protein, 9 aa, synthetic construct
GGTGNDCVD

SEQ ID NO: 23651 - protein, 9 aa, synthetic construct
GGEGNDQIY

SEQ ID NO: 23652 - protein, 9 aa, synthetic construct
GGEGVDTLD

SEQ ID NO: 23653 - protein, 9 aa, synthetic construct
GGTGNDAMW

SEQ ID NO: 23654 - protein, 9 aa, synthetic construct
GGTGNDAML

SEQ ID NO: 23655 - protein, 9 aa, synthetic construct
GGEGVDTLL

SEQ ID NO: 23656 - protein, 9 aa, synthetic construct
GGTGNDALR

SEQ ID NO: 23657 - protein, 9 aa, synthetic construct
GGTGNDALK

SEQ ID NO: 23658 - protein, 9 aa, synthetic construct
GGEGVDTLV

SEQ ID NO: 23659 - protein, 9 aa, synthetic construct
GGTGNDAIF

SEQ ID NO: 23660 - protein, 9 aa, synthetic construct
GGTGNDAID

SEQ ID NO: 23661 - protein, 9 aa, synthetic construct
GGTGNDAFF

SEQ ID NO: 23662 - protein, 9 aa, synthetic construct
GGTGNDAAY

SEQ ID NO: 23663 - protein, 9 aa, synthetic construct
GGTGMDYIS

SEQ ID NO: 23664 - protein, 9 aa, synthetic construct
GGAGFDTFI

SEQ ID NO: 23665 - protein, 9 aa, synthetic construct
GGAGFDTID

SEQ ID NO: 23666 - protein, 9 aa, synthetic construct
GGTGMDTLI

SEQ ID NO: 23667 - protein, 9 aa, synthetic construct
GGTGMDTLF

SEQ ID NO: 23668 - protein, 9 aa, synthetic construct
GGAGFDTIN

SEQ ID NO: 23669 - protein, 9 aa, synthetic construct
GGTGMDTAD

SEQ ID NO: 23670 - protein, 9 aa, synthetic construct
GGAGFDTIV

SEQ ID NO: 23671 - protein, 9 aa, synthetic construct
GGEGVDTAS

SEQ ID NO: 23672 - protein, 9 aa, synthetic construct
GGEGVDTAI

SEQ ID NO: 23673 - protein, 9 aa, synthetic construct
GGTGNDDLV

SEQ ID NO: 23674 - protein, 9 aa, synthetic construct
GGAGFDRLD

SEQ ID NO: 23675 - protein, 9 aa, synthetic construct
GGEGVDRLY

SEQ ID NO: 23676 - protein, 9 aa, synthetic construct
GGTGNDFLT

SEQ ID NO: 23677 - protein, 9 aa, synthetic construct
GGTGNDFLN

SEQ ID NO: 23678 - protein, 9 aa, synthetic construct
GGAGFDQVS

SEQ ID NO: 23679 - protein, 9 aa, synthetic construct
GGTGNDFLH

SEQ ID NO: 23680 - protein, 9 aa, synthetic construct
GGEGNDQLR

SEQ ID NO: 23681 - protein, 9 aa, synthetic construct
GGTGNDFIT

SEQ ID NO: 23682 - protein, 9 aa, synthetic construct
GGAGFDRFI

SEQ ID NO: 23683 - protein, 9 aa, synthetic construct
GGAGFDRFW

SEQ ID NO: 23684 - protein, 9 aa, synthetic construct
GGAGFDRIT

SEQ ID NO: 23685 - protein, 9 aa, synthetic construct
GGEGVDSLF

SEQ ID NO: 23686 - protein, 9 aa, synthetic construct
GGAGFDRLE

SEQ ID NO: 23687 - protein, 9 aa, synthetic construct
GGTGNDDMF

SEQ ID NO: 23688 - protein, 9 aa, synthetic construct
GGAGFDRLI

SEQ ID NO: 23689 - protein, 9 aa, synthetic construct
GGAGFDRLV

SEQ ID NO: 23690 - protein, 9 aa, synthetic construct
GGAGFDRLW

SEQ ID NO: 23691 - protein, 9 aa, synthetic construct
GGAGFDRMH

SEQ ID NO: 23692 - protein, 9 aa, synthetic construct
GGTGNDEID

SEQ ID NO: 23693 - protein, 9 aa, synthetic construct
GGAGFDRMT

SEQ ID NO: 23694 - protein, 9 aa, synthetic construct
GGTGNDEFL

SEQ ID NO: 23695 - protein, 9 aa, synthetic construct
GGAGFDRVA

SEQ ID NO: 23696 - protein, 9 aa, synthetic construct
GGAGFDSFF

SEQ ID NO: 23697 - protein, 9 aa, synthetic construct
GGEGNDQLE

SEQ ID NO: 23698 - protein, 9 aa, synthetic construct
GGTGNDDMH

SEQ ID NO: 23699 - protein, 9 aa, synthetic construct
GGAGFDIAS

SEQ ID NO: 23700 - protein, 9 aa, synthetic construct
GGTGNDLMN

SEQ ID NO: 23701 - protein, 9 aa, synthetic construct
GGTGNDLMT

SEQ ID NO: 23702 - protein, 9 aa, synthetic construct
GGTGNDSII

SEQ ID NO: 23703 - protein, 9 aa, synthetic construct
GGTGNDVIE

SEQ ID NO: 23704 - protein, 9 aa, synthetic construct
GGTGNDVFK

SEQ ID NO: 23705 - protein, 9 aa, synthetic construct
GGAGEDTMF

SEQ ID NO: 23706 - protein, 9 aa, synthetic construct
GGTGNDVAY

SEQ ID NO: 23707 - protein, 9 aa, synthetic construct
GGAGEDTVA

SEQ ID NO: 23708 - protein, 9 aa, synthetic construct
GGTGNDTYM

SEQ ID NO: 23709 - protein, 9 aa, synthetic construct
GGTGNDTVR

SEQ ID NO: 23710 - protein, 9 aa, synthetic construct
GGTGNDTVQ

SEQ ID NO: 23711 - protein, 9 aa, synthetic construct
GGTGNDTVE

SEQ ID NO: 23712 - protein, 9 aa, synthetic construct
GGAGEDTVT

SEQ ID NO: 23713 - protein, 9 aa, synthetic construct
GGTGNDTMK

SEQ ID NO: 23714 - protein, 9 aa, synthetic construct
GGAGEDTVV

SEQ ID NO: 23715 - protein, 9 aa, synthetic construct
GGAGEDVAV

SEQ ID NO: 23716 - protein, 9 aa, synthetic construct
GGTGNDTFT

SEQ ID NO: 23717 - protein, 9 aa, synthetic construct
GGAGEDVFR

SEQ ID NO: 23718 - protein, 9 aa, synthetic construct
GGTGNDTAT

SEQ ID NO: 23719 - protein, 9 aa, synthetic construct
GGAGEDVIH

SEQ ID NO: 23720 - protein, 9 aa, synthetic construct
GGTGNDSYT

SEQ ID NO: 23721 - protein, 9 aa, synthetic construct
GGTGNDSYL

SEQ ID NO: 23722 - protein, 9 aa, synthetic construct
GGAGEDVIR

SEQ ID NO: 23723 - protein, 9 aa, synthetic construct
GGEGTDTMY

SEQ ID NO: 23724 - protein, 9 aa, synthetic construct
GGEGNDRMF

SEQ ID NO: 23725 - protein, 9 aa, synthetic construct
GGTGNDSML

SEQ ID NO: 23726 - protein, 9 aa, synthetic construct
GGTGNDSMF

SEQ ID NO: 23727 - protein, 9 aa, synthetic construct
GGTGNDSIR

SEQ ID NO: 23728 - protein, 9 aa, synthetic construct
GGTGNDVIQ

SEQ ID NO: 23729 - protein, 9 aa, synthetic construct
GGTGNDVIV

SEQ ID NO: 23730 - protein, 9 aa, synthetic construct
GGTGNDVML

SEQ ID NO: 23731 - protein, 9 aa, synthetic construct
GGTGNDWLF

SEQ ID NO: 23732 - protein, 9 aa, synthetic construct
GGTGNDYMG

SEQ ID NO: 23733 - protein, 9 aa, synthetic construct
GGTGNDYMA

SEQ ID NO: 23734 - protein, 9 aa, synthetic construct
GGTGNDYLG

SEQ ID NO: 23735 - protein, 9 aa, synthetic construct
GGAGEDTAS

SEQ ID NO: 23736 - protein, 9 aa, synthetic construct
GGAGEDTAV

SEQ ID NO: 23737 - protein, 9 aa, synthetic construct
GGTGNDYFY

SEQ ID NO: 23738 - protein, 9 aa, synthetic construct
GGAGEDTFL

SEQ ID NO: 23739 - protein, 9 aa, synthetic construct
GGTGNDWVD

SEQ ID NO: 23740 - protein, 9 aa, synthetic construct
GGEGTDTAT

SEQ ID NO: 23741 - protein, 9 aa, synthetic construct
GGAGEDTIE

SEQ ID NO: 23742 - protein, 9 aa, synthetic construct
GGTGNDWLL

SEQ ID NO: 23743 - protein, 9 aa, synthetic construct
GGAGEDTIS

SEQ ID NO: 23744 - protein, 9 aa, synthetic construct
GGTGNDVMV

SEQ ID NO: 23745 - protein, 9 aa, synthetic construct
GGTGNDWIH

SEQ ID NO: 23746 - protein, 9 aa, synthetic construct
GGTGNDWIE

SEQ ID NO: 23747 - protein, 9 aa, synthetic construct
GGEGTDTFI

SEQ ID NO: 23748 - protein, 9 aa, synthetic construct
GGTGNDWFR

SEQ ID NO: 23749 - protein, 9 aa, synthetic construct
GGEGTDTII

SEQ ID NO: 23750 - protein, 9 aa, synthetic construct
GGTGNDVYR

SEQ ID NO: 23751 - protein, 9 aa, synthetic construct
GGTGNDVYL

SEQ ID NO: 23752 - protein, 9 aa, synthetic construct
GGTGNDVVY

SEQ ID NO: 23753 - protein, 9 aa, synthetic construct
GGAGEDTLG

SEQ ID NO: 23754 - protein, 9 aa, synthetic construct
GGTGNDVVL

SEQ ID NO: 23755 - protein, 9 aa, synthetic construct
GGEGTDTIL

SEQ ID NO: 23756 - protein, 9 aa, synthetic construct
GGTGNDSIM

SEQ ID NO: 23757 - protein, 9 aa, synthetic construct
GGTGNDSFS

SEQ ID NO: 23758 - protein, 9 aa, synthetic construct
GGTGNDLVG

SEQ ID NO: 23759 - protein, 9 aa, synthetic construct
GGTGNDSFR

SEQ ID NO: 23760 - protein, 9 aa, synthetic construct
GGTGNDNVN

SEQ ID NO: 23761 - protein, 9 aa, synthetic construct
GGTGNDNMS

SEQ ID NO: 23762 - protein, 9 aa, synthetic construct
GGAGFDDLR

SEQ ID NO: 23763 - protein, 9 aa, synthetic construct
GGAGFDEID

SEQ ID NO: 23764 - protein, 9 aa, synthetic construct
GGTGNDNLL

SEQ ID NO: 23765 - protein, 9 aa, synthetic construct
GGTGNDNLI

SEQ ID NO: 23766 - protein, 9 aa, synthetic construct
GGTGNDNLG

SEQ ID NO: 23767 - protein, 9 aa, synthetic construct
GGTGNDNLA

SEQ ID NO: 23768 - protein, 9 aa, synthetic construct
GGTGNDNIT

SEQ ID NO: 23769 - protein, 9 aa, synthetic construct
GGAGFDFAS

SEQ ID NO: 23770 - protein, 9 aa, synthetic construct
GGEGNDRIV

SEQ ID NO: 23771 - protein, 9 aa, synthetic construct
GGEGNDRIN

SEQ ID NO: 23772 - protein, 9 aa, synthetic construct
GGAGFDGAE

SEQ ID NO: 23773 - protein, 9 aa, synthetic construct
GGTGNDMMF

SEQ ID NO: 23774 - protein, 9 aa, synthetic construct
GGEGVDHYI

SEQ ID NO: 23775 - protein, 9 aa, synthetic construct
GGTGNDMLV

SEQ ID NO: 23776 - protein, 9 aa, synthetic construct
GGEGVDIAS

SEQ ID NO: 23777 - protein, 9 aa, synthetic construct
GGTGNDMLN

SEQ ID NO: 23778 - protein, 9 aa, synthetic construct
GGTGNDMLI

SEQ ID NO: 23779 - protein, 9 aa, synthetic construct
GGEGVDIAV

SEQ ID NO: 23780 - protein, 9 aa, synthetic construct
GGTGNDMLF

SEQ ID NO: 23781 - protein, 9 aa, synthetic construct
GGTGNDMIH

SEQ ID NO: 23782 - protein, 9 aa, synthetic construct
GGTGNDLYQ

SEQ ID NO: 23783 - protein, 9 aa, synthetic construct
GGTGNDLVQ

SEQ ID NO: 23784 - protein, 9 aa, synthetic construct
GGEGVDILL

SEQ ID NO: 23785 - protein, 9 aa, synthetic construct
GGAGFDDID

SEQ ID NO: 23786 - protein, 9 aa, synthetic construct
GGAGFDCVD

SEQ ID NO: 23787 - protein, 9 aa, synthetic construct
GGAGFDAVT

SEQ ID NO: 23788 - protein, 9 aa, synthetic construct
GGTGNDRFL

SEQ ID NO: 23789 - protein, 9 aa, synthetic construct
GGTGNDRYV

SEQ ID NO: 23790 - protein, 9 aa, synthetic construct
GGAGEDVVD

SEQ ID NO: 23791 - protein, 9 aa, synthetic construct
GGAGEDVVF

SEQ ID NO: 23792 - protein, 9 aa, synthetic construct
GGTGNDRVF

SEQ ID NO: 23793 - protein, 9 aa, synthetic construct
GGTGNDRML

SEQ ID NO: 23794 - protein, 9 aa, synthetic construct
GGTGNDRMG

SEQ ID NO: 23795 - protein, 9 aa, synthetic construct
GGTGNDRLG

SEQ ID NO: 23796 - protein, 9 aa, synthetic construct
GGTGNDRIN

SEQ ID NO: 23797 - protein, 9 aa, synthetic construct
GGAGEDWII

SEQ ID NO: 23798 - protein, 9 aa, synthetic construct
GGTGNDRIE

SEQ ID NO: 23799 - protein, 9 aa, synthetic construct
GGEGTDWLA

SEQ ID NO: 23800 - protein, 9 aa, synthetic construct
GGTGNDRFF

SEQ ID NO: 23801 - protein, 9 aa, synthetic construct
GGAGFDAVA

SEQ ID NO: 23802 - protein, 9 aa, synthetic construct
GGEGNDRLK

SEQ ID NO: 23803 - protein, 9 aa, synthetic construct
GGAGEDYLD

SEQ ID NO: 23804 - protein, 9 aa, synthetic construct
GGEGTDYID

SEQ ID NO: 23805 - protein, 9 aa, synthetic construct
GGEGTDYLL

SEQ ID NO: 23806 - protein, 9 aa, synthetic construct
GGTGNDQVW

SEQ ID NO: 23807 - protein, 9 aa, synthetic construct
GGTGNDQVM

SEQ ID NO: 23808 - protein, 9 aa, synthetic construct
GGEGTDYLS

SEQ ID NO: 23809 - protein, 9 aa, synthetic construct
GGTGNDQML

SEQ ID NO: 23810 - protein, 9 aa, synthetic construct
GGEGNDRLH

SEQ ID NO: 23811 - protein, 9 aa, synthetic construct
GGEGVDAIV

SEQ ID NO: 23812 - protein, 9 aa, synthetic construct
GGEGVDALR

SEQ ID NO: 23813 - protein, 9 aa, synthetic construct
GGAGFDTIW

SEQ ID NO: 23814 - protein, 9 aa, synthetic construct
GGTGMDRLL

SEQ ID NO: 23815 - protein, 9 aa, synthetic construct
GGTGMDRLE

SEQ ID NO: 23816 - protein, 9 aa, synthetic construct
GGEGNDLLM

SEQ ID NO: 23817 - protein, 9 aa, synthetic construct
GGTGIDQMH

SEQ ID NO: 23818 - protein, 9 aa, synthetic construct
GGTGIDQLW

SEQ ID NO: 23819 - protein, 9 aa, synthetic construct
GGEGNDLVA

SEQ ID NO: 23820 - protein, 9 aa, synthetic construct
GGTGIDLLR

SEQ ID NO: 23821 - protein, 9 aa, synthetic construct
GGTGIDLLQ

SEQ ID NO: 23822 - protein, 9 aa, synthetic construct
GGTGIDLFV

SEQ ID NO: 23823 - protein, 9 aa, synthetic construct
GGTGIDKLT

SEQ ID NO: 23824 - protein, 9 aa, synthetic construct
GGTGIDKID

SEQ ID NO: 23825 - protein, 9 aa, synthetic construct
GGAGGDLLA

SEQ ID NO: 23826 - protein, 9 aa, synthetic construct
GGTGIDIMY

SEQ ID NO: 23827 - protein, 9 aa, synthetic construct
GGTGIDILT

SEQ ID NO: 23828 - protein, 9 aa, synthetic construct
GGTGIDFLV

SEQ ID NO: 23829 - protein, 9 aa, synthetic construct
GGTGIDELH

SEQ ID NO: 23830 - protein, 9 aa, synthetic construct
GGTGIDEIS

SEQ ID NO: 23831 - protein, 9 aa, synthetic construct
GGTGIDAMT

SEQ ID NO: 23832 - protein, 9 aa, synthetic construct
GGAGGDLMD

SEQ ID NO: 23833 - protein, 9 aa, synthetic construct
GGAGGDLMV

SEQ ID NO: 23834 - protein, 9 aa, synthetic construct
GGAGGDLVE

SEQ ID NO: 23835 - protein, 9 aa, synthetic construct
GGTGIDAFH

SEQ ID NO: 23836 - protein, 9 aa, synthetic construct
GGAGGDLVL

SEQ ID NO: 23837 - protein, 9 aa, synthetic construct
GGTGHDWLG

SEQ ID NO: 23838 - protein, 9 aa, synthetic construct
GGTGHDWLD

SEQ ID NO: 23839 - protein, 9 aa, synthetic construct
GGTGHDVLK

SEQ ID NO: 23840 - protein, 9 aa, synthetic construct
GGTGHDVLH

SEQ ID NO: 23841 - protein, 9 aa, synthetic construct
GGAGGDMLI

SEQ ID NO: 23842 - protein, 9 aa, synthetic construct
GGAGGDKMW

SEQ ID NO: 23843 - protein, 9 aa, synthetic construct
GGTGIDRAL

SEQ ID NO: 23844 - protein, 9 aa, synthetic construct
GGAGGDKLW

SEQ ID NO: 23845 - protein, 9 aa, synthetic construct
GGTGIDTAN

SEQ ID NO: 23846 - protein, 9 aa, synthetic construct
GGEGNDLVV

SEQ ID NO: 23847 - protein, 9 aa, synthetic construct
GGTGIDTMR

SEQ ID NO: 23848 - protein, 9 aa, synthetic construct
GGTGIDTMQ

SEQ ID NO: 23849 - protein, 9 aa, synthetic construct
GGEGNDLVN

SEQ ID NO: 23850 - protein, 9 aa, synthetic construct
GGTGIDTLY

SEQ ID NO: 23851 - protein, 9 aa, synthetic construct
GGTGIDTLK

SEQ ID NO: 23852 - protein, 9 aa, synthetic construct
GGTGIDTLF

SEQ ID NO: 23853 - protein, 9 aa, synthetic construct
GGEGYDTLQ

SEQ ID NO: 23854 - protein, 9 aa, synthetic construct
GGTGIDTFK

SEQ ID NO: 23855 - protein, 9 aa, synthetic construct
GGTGIDTFI

SEQ ID NO: 23856 - protein, 9 aa, synthetic construct
GGTGIDTAT

SEQ ID NO: 23857 - protein, 9 aa, synthetic construct
GGTGIDTAI

SEQ ID NO: 23858 - protein, 9 aa, synthetic construct
GGAGGDKLT

SEQ ID NO: 23859 - protein, 9 aa, synthetic construct
GGAGGDILY

SEQ ID NO: 23860 - protein, 9 aa, synthetic construct
GGAGGDIMI

SEQ ID NO: 23861 - protein, 9 aa, synthetic construct
GGAGGDIMS

SEQ ID NO: 23862 - protein, 9 aa, synthetic construct
GGEGYDTLT

SEQ ID NO: 23863 - protein, 9 aa, synthetic construct
GGAGGDIYV

SEQ ID NO: 23864 - protein, 9 aa, synthetic construct
GGEGYDTLY

SEQ ID NO: 23865 - protein, 9 aa, synthetic construct
GGAGGDKFF

SEQ ID NO: 23866 - protein, 9 aa, synthetic construct
GGEGYDTVR

SEQ ID NO: 23867 - protein, 9 aa, synthetic construct
GGAGGDKLA

SEQ ID NO: 23868 - protein, 9 aa, synthetic construct
GGTGIDRMI

SEQ ID NO: 23869 - protein, 9 aa, synthetic construct
GGAGGDKLE

SEQ ID NO: 23870 - protein, 9 aa, synthetic construct
GGTGHDVLD

SEQ ID NO: 23871 - protein, 9 aa, synthetic construct
GGAGGDNFI

SEQ ID NO: 23872 - protein, 9 aa, synthetic construct
GGAGGDIIN

SEQ ID NO: 23873 - protein, 9 aa, synthetic construct
GGTGHDTVN

SEQ ID NO: 23874 - protein, 9 aa, synthetic construct
GGAGGDRLQ

SEQ ID NO: 23875 - protein, 9 aa, synthetic construct
GGTGHDFLD

SEQ ID NO: 23876 - protein, 9 aa, synthetic construct
GGTGHDELY

SEQ ID NO: 23877 - protein, 9 aa, synthetic construct
GGTGHDEIQ

SEQ ID NO: 23878 - protein, 9 aa, synthetic construct
GGAGGDRLY

SEQ ID NO: 23879 - protein, 9 aa, synthetic construct
GGEGNDLIN

SEQ ID NO: 23880 - protein, 9 aa, synthetic construct
GGEGNDLII

SEQ ID NO: 23881 - protein, 9 aa, synthetic construct
GGEGNDLIG

SEQ ID NO: 23882 - protein, 9 aa, synthetic construct
GGAGGDRMS

SEQ ID NO: 23883 - protein, 9 aa, synthetic construct
GGFGADGIH

SEQ ID NO: 23884 - protein, 9 aa, synthetic construct
GGAGGDRYV

SEQ ID NO: 23885 - protein, 9 aa, synthetic construct
GGTGGDYME

SEQ ID NO: 23886 - protein, 9 aa, synthetic construct
GGTGGDYLY

SEQ ID NO: 23887 - protein, 9 aa, synthetic construct
GGAGGDSFD

SEQ ID NO: 23888 - protein, 9 aa, synthetic construct
GGTGGDYIS

SEQ ID NO: 23889 - protein, 9 aa, synthetic construct
GGTGGDWLN

SEQ ID NO: 23890 - protein, 9 aa, synthetic construct
GGTGGDWIE

SEQ ID NO: 23891 - protein, 9 aa, synthetic construct
GGTGGDVMQ

SEQ ID NO: 23892 - protein, 9 aa, synthetic construct
GGFGADIFV

SEQ ID NO: 23893 - protein, 9 aa, synthetic construct
GGFGADILA

SEQ ID NO: 23894 - protein, 9 aa, synthetic construct
GGAGGDSLN

SEQ ID NO: 23895 - protein, 9 aa, synthetic construct
GGTGGDVLI

SEQ ID NO: 23896 - protein, 9 aa, synthetic construct
GGTGGDVIN

SEQ ID NO: 23897 - protein, 9 aa, synthetic construct
GGTGGDVFV

SEQ ID NO: 23898 - protein, 9 aa, synthetic construct
GGTGGDTYI

SEQ ID NO: 23899 - protein, 9 aa, synthetic construct
GGAGGDRLN

SEQ ID NO: 23900 - protein, 9 aa, synthetic construct
GGAGGDRLM

SEQ ID NO: 23901 - protein, 9 aa, synthetic construct
GGAGGDRLA

SEQ ID NO: 23902 - protein, 9 aa, synthetic construct
GGAGGDQLD

SEQ ID NO: 23903 - protein, 9 aa, synthetic construct
GGAGGDNLA

SEQ ID NO: 23904 - protein, 9 aa, synthetic construct
GGTGHDTMN

SEQ ID NO: 23905 - protein, 9 aa, synthetic construct
GGTGHDTMH

SEQ ID NO: 23906 - protein, 9 aa, synthetic construct
GGTGHDTLH

SEQ ID NO: 23907 - protein, 9 aa, synthetic construct
GGTGHDTIR

SEQ ID NO: 23908 - protein, 9 aa, synthetic construct
GGAGGDNLL

SEQ ID NO: 23909 - protein, 9 aa, synthetic construct
GGTGHDTII

SEQ ID NO: 23910 - protein, 9 aa, synthetic construct
GGTGHDTAV

SEQ ID NO: 23911 - protein, 9 aa, synthetic construct
GGTGHDTAS

SEQ ID NO: 23912 - protein, 9 aa, synthetic construct
GGAGGDNLW

SEQ ID NO: 23913 - protein, 9 aa, synthetic construct
GGTGHDSLW

SEQ ID NO: 23914 - protein, 9 aa, synthetic construct
GGTGHDRYR

SEQ ID NO: 23915 - protein, 9 aa, synthetic construct
GGTGHDLFE

SEQ ID NO: 23916 - protein, 9 aa, synthetic construct
GGTGHDRLT

SEQ ID NO: 23917 - protein, 9 aa, synthetic construct
GGAGGDQLT

SEQ ID NO: 23918 - protein, 9 aa, synthetic construct
GGEGNDLIV

SEQ ID NO: 23919 - protein, 9 aa, synthetic construct
GGEGNDLIS

SEQ ID NO: 23920 - protein, 9 aa, synthetic construct
GGFGADELH

SEQ ID NO: 23921 - protein, 9 aa, synthetic construct
GGTGHDQLF

SEQ ID NO: 23922 - protein, 9 aa, synthetic construct
GGTGHDQIS

SEQ ID NO: 23923 - protein, 9 aa, synthetic construct
GGAGGDRFF

SEQ ID NO: 23924 - protein, 9 aa, synthetic construct
GGFGADELV

SEQ ID NO: 23925 - protein, 9 aa, synthetic construct
GGTGHDLLY

SEQ ID NO: 23926 - protein, 9 aa, synthetic construct
GGTGHDLLV

SEQ ID NO: 23927 - protein, 9 aa, synthetic construct
GGTGIDTVS

SEQ ID NO: 23928 - protein, 9 aa, synthetic construct
GGTGIDVAL

SEQ ID NO: 23929 - protein, 9 aa, synthetic construct
GGTGMDQLY

SEQ ID NO: 23930 - protein, 9 aa, synthetic construct
GGAGGDAFV

SEQ ID NO: 23931 - protein, 9 aa, synthetic construct
GGTGLDMLY

SEQ ID NO: 23932 - protein, 9 aa, synthetic construct
GGEGNDNLR

SEQ ID NO: 23933 - protein, 9 aa, synthetic construct
GGTGLDLLL

SEQ ID NO: 23934 - protein, 9 aa, synthetic construct
GGTGLDLLF

SEQ ID NO: 23935 - protein, 9 aa, synthetic construct
GGEGVDYLI

SEQ ID NO: 23936 - protein, 9 aa, synthetic construct
GGAGFDVVT

SEQ ID NO: 23937 - protein, 9 aa, synthetic construct
GGAGFDVYK

SEQ ID NO: 23938 - protein, 9 aa, synthetic construct
GGAGFDWAD

SEQ ID NO: 23939 - protein, 9 aa, synthetic construct
GGAGFDWLD

SEQ ID NO: 23940 - protein, 9 aa, synthetic construct
GGEGWDAIL

SEQ ID NO: 23941 - protein, 9 aa, synthetic construct
GGAGFDWLI

SEQ ID NO: 23942 - protein, 9 aa, synthetic construct
GGTGLDHLS

SEQ ID NO: 23943 - protein, 9 aa, synthetic construct
GGTGLDFLY

SEQ ID NO: 23944 - protein, 9 aa, synthetic construct
GGTGLDFLT

SEQ ID NO: 23945 - protein, 9 aa, synthetic construct
GGEGNDNLL

SEQ ID NO: 23946 - protein, 9 aa, synthetic construct
GGAGFDWVD

SEQ ID NO: 23947 - protein, 9 aa, synthetic construct
GGAGFDWVV

SEQ ID NO: 23948 - protein, 9 aa, synthetic construct
GGEGWDILT

SEQ ID NO: 23949 - protein, 9 aa, synthetic construct
GGAGFDYLD

SEQ ID NO: 23950 - protein, 9 aa, synthetic construct
GGAGFDYLF

SEQ ID NO: 23951 - protein, 9 aa, synthetic construct
GGTGKDYLH

SEQ ID NO: 23952 - protein, 9 aa, synthetic construct
GGEGNDNLG

SEQ ID NO: 23953 - protein, 9 aa, synthetic construct
GGEGWDQLF

SEQ ID NO: 23954 - protein, 9 aa, synthetic construct
GGTGKDVMV

SEQ ID NO: 23955 - protein, 9 aa, synthetic construct
GGAGFDYME

SEQ ID NO: 23956 - protein, 9 aa, synthetic construct
GGAGFDVLI

SEQ ID NO: 23957 - protein, 9 aa, synthetic construct
GGAGFDVLF

SEQ ID NO: 23958 - protein, 9 aa, synthetic construct
GGTGLDRAE

SEQ ID NO: 23959 - protein, 9 aa, synthetic construct
GGTGLDTLY

SEQ ID NO: 23960 - protein, 9 aa, synthetic construct
GGTGMDQLF

SEQ ID NO: 23961 - protein, 9 aa, synthetic construct
GGTGMDIFV

SEQ ID NO: 23962 - protein, 9 aa, synthetic construct
GGAGFDTLH

SEQ ID NO: 23963 - protein, 9 aa, synthetic construct
GGEGVDTYT

SEQ ID NO: 23964 - protein, 9 aa, synthetic construct
GGEGNDQIE

SEQ ID NO: 23965 - protein, 9 aa, synthetic construct
GGTGLDWMI

SEQ ID NO: 23966 - protein, 9 aa, synthetic construct
GGTGLDVLT

SEQ ID NO: 23967 - protein, 9 aa, synthetic construct
GGTGLDVLF

SEQ ID NO: 23968 - protein, 9 aa, synthetic construct
GGEGNDQFR

SEQ ID NO: 23969 - protein, 9 aa, synthetic construct
GGTGLDTVD

SEQ ID NO: 23970 - protein, 9 aa, synthetic construct
GGTGLDTMT

SEQ ID NO: 23971 - protein, 9 aa, synthetic construct
GGAGFDTVM

SEQ ID NO: 23972 - protein, 9 aa, synthetic construct
GGAGFDVLD

SEQ ID NO: 23973 - protein, 9 aa, synthetic construct
GGAGFDTVW

SEQ ID NO: 23974 - protein, 9 aa, synthetic construct
GGAGFDTYR

SEQ ID NO: 23975 - protein, 9 aa, synthetic construct
GGAGFDVAD

SEQ ID NO: 23976 - protein, 9 aa, synthetic construct
GGEGVDVLS

SEQ ID NO: 23977 - protein, 9 aa, synthetic construct
GGAGFDVAT

SEQ ID NO: 23978 - protein, 9 aa, synthetic construct
GGTGLDRMT

SEQ ID NO: 23979 - protein, 9 aa, synthetic construct
GGTGLDRLV

SEQ ID NO: 23980 - protein, 9 aa, synthetic construct
GGEGVDWIY

SEQ ID NO: 23981 - protein, 9 aa, synthetic construct
GGTGLDRLN

SEQ ID NO: 23982 - protein, 9 aa, synthetic construct
GGAGFDVID

SEQ ID NO: 23983 - protein, 9 aa, synthetic construct
GGTGLDRLA

SEQ ID NO: 23984 - protein, 9 aa, synthetic construct
GGAGGDAFN

SEQ ID NO: 23985 - protein, 9 aa, synthetic construct
GGTGKDVLS

SEQ ID NO: 23986 - protein, 9 aa, synthetic construct
GGAGGDIII

SEQ ID NO: 23987 - protein, 9 aa, synthetic construct
GGTGKDVLA

SEQ ID NO: 23988 - protein, 9 aa, synthetic construct
GGAGGDELC

SEQ ID NO: 23989 - protein, 9 aa, synthetic construct
GGTGKDQLW

SEQ ID NO: 23990 - protein, 9 aa, synthetic construct
GGTGKDQLF

SEQ ID NO: 23991 - protein, 9 aa, synthetic construct
GGTGKDNLT

SEQ ID NO: 23992 - protein, 9 aa, synthetic construct
GGEGYDIID

SEQ ID NO: 23993 - protein, 9 aa, synthetic construct
GGTGKDMLN

SEQ ID NO: 23994 - protein, 9 aa, synthetic construct
GGTGKDLMY

SEQ ID NO: 23995 - protein, 9 aa, synthetic construct
GGEGNDMLR

SEQ ID NO: 23996 - protein, 9 aa, synthetic construct
GGTGKDLLS

SEQ ID NO: 23997 - protein, 9 aa, synthetic construct
GGTGKDLLK

SEQ ID NO: 23998 - protein, 9 aa, synthetic construct
GGTGKDLLE

SEQ ID NO: 23999 - protein, 9 aa, synthetic construct
GGAGGDFIA

SEQ ID NO: 24000 - protein, 9 aa, synthetic construct
GGTGKDKLR

SEQ ID NO: 24001 - protein, 9 aa, synthetic construct
GGEGYDLLR

SEQ ID NO: 24002 - protein, 9 aa, synthetic construct
GGTGKDHLY

SEQ ID NO: 24003 - protein, 9 aa, synthetic construct
GGEGNDMIH

SEQ ID NO: 24004 - protein, 9 aa, synthetic construct
GGEGNDMFV

SEQ ID NO: 24005 - protein, 9 aa, synthetic construct
GGTGKDFLL

SEQ ID NO: 24006 - protein, 9 aa, synthetic construct
GGAGGDHLE

SEQ ID NO: 24007 - protein, 9 aa, synthetic construct
GGTGKDALT

SEQ ID NO: 24008 - protein, 9 aa, synthetic construct
GGEGYDTAV

SEQ ID NO: 24009 - protein, 9 aa, synthetic construct
GGTGIDVMS

SEQ ID NO: 24010 - protein, 9 aa, synthetic construct
GGAGGDIFR

SEQ ID NO: 24011 - protein, 9 aa, synthetic construct
GGAGGDIID

SEQ ID NO: 24012 - protein, 9 aa, synthetic construct
GGTGIDVLI

SEQ ID NO: 24013 - protein, 9 aa, synthetic construct
GGEGNDNFD

SEQ ID NO: 24014 - protein, 9 aa, synthetic construct
GGTGKDRLY

SEQ ID NO: 24015 - protein, 9 aa, synthetic construct
GGTGKDRMD

SEQ ID NO: 24016 - protein, 9 aa, synthetic construct
GGTGKDTLH

SEQ ID NO: 24017 - protein, 9 aa, synthetic construct
GGEGNDNIV

SEQ ID NO: 24018 - protein, 9 aa, synthetic construct
GGTGKDVFN

SEQ ID NO: 24019 - protein, 9 aa, synthetic construct
GGEGWDVLF

SEQ ID NO: 24020 - protein, 9 aa, synthetic construct
GGEGWDVLH

SEQ ID NO: 24021 - protein, 9 aa, synthetic construct
GGAGGDALN

SEQ ID NO: 24022 - protein, 9 aa, synthetic construct
GGAGGDALR

SEQ ID NO: 24023 - protein, 9 aa, synthetic construct
GGAGGDALS

SEQ ID NO: 24024 - protein, 9 aa, synthetic construct
GGEGNDNIS

SEQ ID NO: 24025 - protein, 9 aa, synthetic construct
GGTGKDTMT

SEQ ID NO: 24026 - protein, 9 aa, synthetic construct
GGAGGDAMD

SEQ ID NO: 24027 - protein, 9 aa, synthetic construct
GGTGKDTLY

SEQ ID NO: 24028 - protein, 9 aa, synthetic construct
GGAGGDAMW

SEQ ID NO: 24029 - protein, 9 aa, synthetic construct
GGAGGDDLW

SEQ ID NO: 24030 - protein, 9 aa, synthetic construct
GGTGKDTFL

SEQ ID NO: 24031 - protein, 9 aa, synthetic construct
GGTGKDTFK

SEQ ID NO: 24032 - protein, 9 aa, synthetic construct
GGAGGDDFD

SEQ ID NO: 24033 - protein, 9 aa, synthetic construct
GGAGGDDIA

SEQ ID NO: 24034 - protein, 9 aa, synthetic construct
GGAGGDDIT

SEQ ID NO: 24035 - protein, 9 aa, synthetic construct
GGTGKDSLY

SEQ ID NO: 24036 - protein, 9 aa, synthetic construct
GGTGKDSLV

SEQ ID NO: 24037 - protein, 9 aa, synthetic construct
GGTGKDSLT

SEQ ID NO: 24038 - protein, 9 aa, synthetic construct
GGTGKDSLF

SEQ ID NO: 24039 - protein, 9 aa, synthetic construct
GGAGGDDLR

SEQ ID NO: 24040 - protein, 9 aa, synthetic construct
GGTGKDSFQ

SEQ ID NO: 24041 - protein, 9 aa, synthetic construct
GGTGNDYMI

SEQ ID NO: 24042 - protein, 9 aa, synthetic construct
GGEGTDSVS

SEQ ID NO: 24043 - protein, 9 aa, synthetic construct
GGTGNDYVY

SEQ ID NO: 24044 - protein, 9 aa, synthetic construct
GGTGTDIMR

SEQ ID NO: 24045 - protein, 9 aa, synthetic construct
GGTGTDTLE

SEQ ID NO: 24046 - protein, 9 aa, synthetic construct
GGTGTDTIN

SEQ ID NO: 24047 - protein, 9 aa, synthetic construct
GGTGTDTFD

SEQ ID NO: 24048 - protein, 9 aa, synthetic construct
GGAGDDTIK

SEQ ID NO: 24049 - protein, 9 aa, synthetic construct
GGTGTDSMD

SEQ ID NO: 24050 - protein, 9 aa, synthetic construct
GGTGTDSLY

SEQ ID NO: 24051 - protein, 9 aa, synthetic construct
GGTGTDSLV

SEQ ID NO: 24052 - protein, 9 aa, synthetic construct
GGTGTDSID

SEQ ID NO: 24053 - protein, 9 aa, synthetic construct
GGEGSDTYE

SEQ ID NO: 24054 - protein, 9 aa, synthetic construct
GGTGTDRLV

SEQ ID NO: 24055 - protein, 9 aa, synthetic construct
GGTGTDRLL

SEQ ID NO: 24056 - protein, 9 aa, synthetic construct
GGTGTDRIS

SEQ ID NO: 24057 - protein, 9 aa, synthetic construct
GGTGTDRAS

SEQ ID NO: 24058 - protein, 9 aa, synthetic construct
GGTGTDQLY

SEQ ID NO: 24059 - protein, 9 aa, synthetic construct
GGTGTDNVS

SEQ ID NO: 24060 - protein, 9 aa, synthetic construct
GGTGTDNVD

SEQ ID NO: 24061 - protein, 9 aa, synthetic construct
GGTGTDNLS

SEQ ID NO: 24062 - protein, 9 aa, synthetic construct
GGTGTDNLQ

SEQ ID NO: 24063 - protein, 9 aa, synthetic construct
GGAGDDTMH

SEQ ID NO: 24064 - protein, 9 aa, synthetic construct
GGTGTDMAF

SEQ ID NO: 24065 - protein, 9 aa, synthetic construct
GGAGDDTMQ

SEQ ID NO: 24066 - protein, 9 aa, synthetic construct
GGTGTDLLF

SEQ ID NO: 24067 - protein, 9 aa, synthetic construct
GGTGTDLIN

SEQ ID NO: 24068 - protein, 9 aa, synthetic construct
GGTGTDLID

SEQ ID NO: 24069 - protein, 9 aa, synthetic construct
GGTGTDKLS

SEQ ID NO: 24070 - protein, 9 aa, synthetic construct
GGTGTDTLL

SEQ ID NO: 24071 - protein, 9 aa, synthetic construct
GGTGTDTLN

SEQ ID NO: 24072 - protein, 9 aa, synthetic construct
GGAGDDTFQ

SEQ ID NO: 24073 - protein, 9 aa, synthetic construct
GGAGDDSYF

SEQ ID NO: 24074 - protein, 9 aa, synthetic construct
GGTGVDKMT

SEQ ID NO: 24075 - protein, 9 aa, synthetic construct
GGAGDDSMN

SEQ ID NO: 24076 - protein, 9 aa, synthetic construct
GGTGVDKMN

SEQ ID NO: 24077 - protein, 9 aa, synthetic construct
GGEGSDTLQ

SEQ ID NO: 24078 - protein, 9 aa, synthetic construct
GGAGDDSMS

SEQ ID NO: 24079 - protein, 9 aa, synthetic construct
GGAGDDSMV

SEQ ID NO: 24080 - protein, 9 aa, synthetic construct
GGTGVDILL

SEQ ID NO: 24081 - protein, 9 aa, synthetic construct
GGAGDDSVI

SEQ ID NO: 24082 - protein, 9 aa, synthetic construct
GGEGSDTML

SEQ ID NO: 24083 - protein, 9 aa, synthetic construct
GGAGDDSVQ

SEQ ID NO: 24084 - protein, 9 aa, synthetic construct
GGAGDDSYD

SEQ ID NO: 24085 - protein, 9 aa, synthetic construct
GGEGSDTVE

SEQ ID NO: 24086 - protein, 9 aa, synthetic construct
GGTGTDTMR

SEQ ID NO: 24087 - protein, 9 aa, synthetic construct
GGTGTDYLN

SEQ ID NO: 24088 - protein, 9 aa, synthetic construct
GGAGDDTAH

SEQ ID NO: 24089 - protein, 9 aa, synthetic construct
GGAGDDTAI

SEQ ID NO: 24090 - protein, 9 aa, synthetic construct
GGTGTDWFV

SEQ ID NO: 24091 - protein, 9 aa, synthetic construct
GGTGTDVVT

SEQ ID NO: 24092 - protein, 9 aa, synthetic construct
GGEGNDTFL

SEQ ID NO: 24093 - protein, 9 aa, synthetic construct
GGTGTDVLS

SEQ ID NO: 24094 - protein, 9 aa, synthetic construct
GGTGTDVLA

SEQ ID NO: 24095 - protein, 9 aa, synthetic construct
GGTGTDVII

SEQ ID NO: 24096 - protein, 9 aa, synthetic construct
GGAGDDTFG

SEQ ID NO: 24097 - protein, 9 aa, synthetic construct
GGTGTDTMT

SEQ ID NO: 24098 - protein, 9 aa, synthetic construct
GGTGTDIMT

SEQ ID NO: 24099 - protein, 9 aa, synthetic construct
GGAGDDTVH

SEQ ID NO: 24100 - protein, 9 aa, synthetic construct
GGAGDDSMH

SEQ ID NO: 24101 - protein, 9 aa, synthetic construct
GGTGTDIFA

SEQ ID NO: 24102 - protein, 9 aa, synthetic construct
GGAGDDVFN

SEQ ID NO: 24103 - protein, 9 aa, synthetic construct
GGAGDDVFS

SEQ ID NO: 24104 - protein, 9 aa, synthetic construct
GGTGSDTMS

SEQ ID NO: 24105 - protein, 9 aa, synthetic construct
GGEGSDVAV

SEQ ID NO: 24106 - protein, 9 aa, synthetic construct
GGTGSDTFM

SEQ ID NO: 24107 - protein, 9 aa, synthetic construct
GGTGSDTFL

SEQ ID NO: 24108 - protein, 9 aa, synthetic construct
GGAGDDVLC

SEQ ID NO: 24109 - protein, 9 aa, synthetic construct
GGTGSDTAW

SEQ ID NO: 24110 - protein, 9 aa, synthetic construct
GGTGSDTAT

SEQ ID NO: 24111 - protein, 9 aa, synthetic construct
GGTGSDSVY

SEQ ID NO: 24112 - protein, 9 aa, synthetic construct
GGTGSDSMT

SEQ ID NO: 24113 - protein, 9 aa, synthetic construct
GGTGSDSLV

SEQ ID NO: 24114 - protein, 9 aa, synthetic construct
GGTGSDSLR

SEQ ID NO: 24115 - protein, 9 aa, synthetic construct
GGTGSDSLL

SEQ ID NO: 24116 - protein, 9 aa, synthetic construct
GGTGSDSLE

SEQ ID NO: 24117 - protein, 9 aa, synthetic construct
GGTGSDSIN

SEQ ID NO: 24118 - protein, 9 aa, synthetic construct
GGTGSDSIL

SEQ ID NO: 24119 - protein, 9 aa, synthetic construct
GGTGSDSIA

SEQ ID NO: 24120 - protein, 9 aa, synthetic construct
GGTGSDSFV

SEQ ID NO: 24121 - protein, 9 aa, synthetic construct
GGTGSDRVT

SEQ ID NO: 24122 - protein, 9 aa, synthetic construct
GGTGSDRMY

SEQ ID NO: 24123 - protein, 9 aa, synthetic construct
GGTGSDRMT

SEQ ID NO: 24124 - protein, 9 aa, synthetic construct
GGTGSDRLT

SEQ ID NO: 24125 - protein, 9 aa, synthetic construct
GGTGSDRLS

SEQ ID NO: 24126 - protein, 9 aa, synthetic construct
GGTGSDRLR

SEQ ID NO: 24127 - protein, 9 aa, synthetic construct
GGTGSDVLA

SEQ ID NO: 24128 - protein, 9 aa, synthetic construct
GGTGSDVLE

SEQ ID NO: 24129 - protein, 9 aa, synthetic construct
GGTGSDVLL

SEQ ID NO: 24130 - protein, 9 aa, synthetic construct
GGTGTDAAL

SEQ ID NO: 24131 - protein, 9 aa, synthetic construct
GGTGTDIAD

SEQ ID NO: 24132 - protein, 9 aa, synthetic construct
GGEGNDTFH

SEQ ID NO: 24133 - protein, 9 aa, synthetic construct
GGTGTDHLE

SEQ ID NO: 24134 - protein, 9 aa, synthetic construct
GGAGDDTVQ

SEQ ID NO: 24135 - protein, 9 aa, synthetic construct
GGTGTDFVT

SEQ ID NO: 24136 - protein, 9 aa, synthetic construct
GGTGTDFLY

SEQ ID NO: 24137 - protein, 9 aa, synthetic construct
GGTGTDFLT

SEQ ID NO: 24138 - protein, 9 aa, synthetic construct
GGTGTDFAS

SEQ ID NO: 24139 - protein, 9 aa, synthetic construct
GGTGTDDLR

SEQ ID NO: 24140 - protein, 9 aa, synthetic construct
GGTGTDALF

SEQ ID NO: 24141 - protein, 9 aa, synthetic construct
GGTGTDAAV

SEQ ID NO: 24142 - protein, 9 aa, synthetic construct
GGAGDDTYN

SEQ ID NO: 24143 - protein, 9 aa, synthetic construct
GGTGSDVMD

SEQ ID NO: 24144 - protein, 9 aa, synthetic construct
GGAGDDTYP

SEQ ID NO: 24145 - protein, 9 aa, synthetic construct
GGTGSDYLT

SEQ ID NO: 24146 - protein, 9 aa, synthetic construct
GGAGDDVAD

SEQ ID NO: 24147 - protein, 9 aa, synthetic construct
GGTGSDWLT

SEQ ID NO: 24148 - protein, 9 aa, synthetic construct
GGTGSDWLR

SEQ ID NO: 24149 - protein, 9 aa, synthetic construct
GGAGDDVAI

SEQ ID NO: 24150 - protein, 9 aa, synthetic construct
GGAGDDVAQ

SEQ ID NO: 24151 - protein, 9 aa, synthetic construct
GGTGSDWIE

SEQ ID NO: 24152 - protein, 9 aa, synthetic construct
GGAGDDVAR

SEQ ID NO: 24153 - protein, 9 aa, synthetic construct
GGAGDDVFD

SEQ ID NO: 24154 - protein, 9 aa, synthetic construct
GGEGSDTYT

SEQ ID NO: 24155 - protein, 9 aa, synthetic construct
GGAGDDSMI

SEQ ID NO: 24156 - protein, 9 aa, synthetic construct
GGTGVDLLD

SEQ ID NO: 24157 - protein, 9 aa, synthetic construct
GGAGDDVMA

SEQ ID NO: 24158 - protein, 9 aa, synthetic construct
GGEGSDTFW

SEQ ID NO: 24159 - protein, 9 aa, synthetic construct
GGVGADNLS

SEQ ID NO: 24160 - protein, 9 aa, synthetic construct
GGVGADNLQ

SEQ ID NO: 24161 - protein, 9 aa, synthetic construct
GGVGADNLI

SEQ ID NO: 24162 - protein, 9 aa, synthetic construct
GGVGADNAN

SEQ ID NO: 24163 - protein, 9 aa, synthetic construct
GGVGADMLT

SEQ ID NO: 24164 - protein, 9 aa, synthetic construct
GGVGADMLI

SEQ ID NO: 24165 - protein, 9 aa, synthetic construct
GGVGADLVQ

SEQ ID NO: 24166 - protein, 9 aa, synthetic construct
GGVGADLMV

SEQ ID NO: 24167 - protein, 9 aa, synthetic construct
GGVGADLMT

SEQ ID NO: 24168 - protein, 9 aa, synthetic construct
GGEGSDSVY

SEQ ID NO: 24169 - protein, 9 aa, synthetic construct
GGEGSDSYW

SEQ ID NO: 24170 - protein, 9 aa, synthetic construct
GGVGADLLY

SEQ ID NO: 24171 - protein, 9 aa, synthetic construct
GGAGDDQMH

SEQ ID NO: 24172 - protein, 9 aa, synthetic construct
GGEGSDTAI

SEQ ID NO: 24173 - protein, 9 aa, synthetic construct
GGVGADLLE

SEQ ID NO: 24174 - protein, 9 aa, synthetic construct
GGAGDDQMV

SEQ ID NO: 24175 - protein, 9 aa, synthetic construct
GGAGDDQVE

SEQ ID NO: 24176 - protein, 9 aa, synthetic construct
GGAGDDQVF

SEQ ID NO: 24177 - protein, 9 aa, synthetic construct
GGAGDDQVL

SEQ ID NO: 24178 - protein, 9 aa, synthetic construct
GGVGADIMS

SEQ ID NO: 24179 - protein, 9 aa, synthetic construct
GGVGADIMR

SEQ ID NO: 24180 - protein, 9 aa, synthetic construct
GGVGADIMI

SEQ ID NO: 24181 - protein, 9 aa, synthetic construct
GGAGDDQVQ

SEQ ID NO: 24182 - protein, 9 aa, synthetic construct
GGEGSDTAY

SEQ ID NO: 24183 - protein, 9 aa, synthetic construct
GGVGADILF

SEQ ID NO: 24184 - protein, 9 aa, synthetic construct
GGVGADNLT

SEQ ID NO: 24185 - protein, 9 aa, synthetic construct
GGVGADNMK

SEQ ID NO: 24186 - protein, 9 aa, synthetic construct
GGVGADQFV

SEQ ID NO: 24187 - protein, 9 aa, synthetic construct
GGVGADTAV

SEQ ID NO: 24188 - protein, 9 aa, synthetic construct
GGVGADTVI

SEQ ID NO: 24189 - protein, 9 aa, synthetic construct
GGEGSDSLT

SEQ ID NO: 24190 - protein, 9 aa, synthetic construct
GGAGDDQFA

SEQ ID NO: 24191 - protein, 9 aa, synthetic construct
GGAGDDQFT

SEQ ID NO: 24192 - protein, 9 aa, synthetic construct
GGVGADTLQ

SEQ ID NO: 24193 - protein, 9 aa, synthetic construct
GGEGSDSMF

SEQ ID NO: 24194 - protein, 9 aa, synthetic construct
GGVGADTIE

SEQ ID NO: 24195 - protein, 9 aa, synthetic construct
GGVGADTID

SEQ ID NO: 24196 - protein, 9 aa, synthetic construct
GGVGADTFQ

SEQ ID NO: 24197 - protein, 9 aa, synthetic construct
GGVGADTFI

SEQ ID NO: 24198 - protein, 9 aa, synthetic construct
GGVGADTFF

SEQ ID NO: 24199 - protein, 9 aa, synthetic construct
GGVGADSYH

SEQ ID NO: 24200 - protein, 9 aa, synthetic construct
GGVGADQIR

SEQ ID NO: 24201 - protein, 9 aa, synthetic construct
GGAGDDQIH

SEQ ID NO: 24202 - protein, 9 aa, synthetic construct
GGAGDDQII

SEQ ID NO: 24203 - protein, 9 aa, synthetic construct
GGEGSDSVF

SEQ ID NO: 24204 - protein, 9 aa, synthetic construct
GGVGADSLV

SEQ ID NO: 24205 - protein, 9 aa, synthetic construct
GGVGADSFV

SEQ ID NO: 24206 - protein, 9 aa, synthetic construct
GGAGDDQIY

SEQ ID NO: 24207 - protein, 9 aa, synthetic construct
GGVGADRMY

SEQ ID NO: 24208 - protein, 9 aa, synthetic construct
GGVGADRMT

SEQ ID NO: 24209 - protein, 9 aa, synthetic construct
GGVGADRII

SEQ ID NO: 24210 - protein, 9 aa, synthetic construct
GGVGADRID

SEQ ID NO: 24211 - protein, 9 aa, synthetic construct
GGAGDDQLG

SEQ ID NO: 24212 - protein, 9 aa, synthetic construct
GGAGDDQYI

SEQ ID NO: 24213 - protein, 9 aa, synthetic construct
GGVGADGLF

SEQ ID NO: 24214 - protein, 9 aa, synthetic construct
GGTGVDLVI

SEQ ID NO: 24215 - protein, 9 aa, synthetic construct
GGAGDDRFI

SEQ ID NO: 24216 - protein, 9 aa, synthetic construct
GGAGDDRYQ

SEQ ID NO: 24217 - protein, 9 aa, synthetic construct
GGTGVDYLT

SEQ ID NO: 24218 - protein, 9 aa, synthetic construct
GGAGDDRYR

SEQ ID NO: 24219 - protein, 9 aa, synthetic construct
GGTGVDYLE

SEQ ID NO: 24220 - protein, 9 aa, synthetic construct
GGAGDDRYY

SEQ ID NO: 24221 - protein, 9 aa, synthetic construct
GGTGVDVVR

SEQ ID NO: 24222 - protein, 9 aa, synthetic construct
GGAGDDSFA

SEQ ID NO: 24223 - protein, 9 aa, synthetic construct
GGTGVDVLT

SEQ ID NO: 24224 - protein, 9 aa, synthetic construct
GGAGDDSFH

SEQ ID NO: 24225 - protein, 9 aa, synthetic construct
GGTGVDVLM

SEQ ID NO: 24226 - protein, 9 aa, synthetic construct
GGTGVDVID

SEQ ID NO: 24227 - protein, 9 aa, synthetic construct
GGTGVDTYV

SEQ ID NO: 24228 - protein, 9 aa, synthetic construct
GGTGVDTMY

SEQ ID NO: 24229 - protein, 9 aa, synthetic construct
GGTGVDTLS

SEQ ID NO: 24230 - protein, 9 aa, synthetic construct
GGTGVDTLL

SEQ ID NO: 24231 - protein, 9 aa, synthetic construct
GGTGVDTIH

SEQ ID NO: 24232 - protein, 9 aa, synthetic construct
GGTGVDTFV

SEQ ID NO: 24233 - protein, 9 aa, synthetic construct
GGTGVDTAS

SEQ ID NO: 24234 - protein, 9 aa, synthetic construct
GGTGVDSLL

SEQ ID NO: 24235 - protein, 9 aa, synthetic construct
GGEGSDTLM

SEQ ID NO: 24236 - protein, 9 aa, synthetic construct
GGTGVDRLN

SEQ ID NO: 24237 - protein, 9 aa, synthetic construct
GGTGVDRLE

SEQ ID NO: 24238 - protein, 9 aa, synthetic construct
GGTGVDRAF

SEQ ID NO: 24239 - protein, 9 aa, synthetic construct
GGTGVDQLY

SEQ ID NO: 24240 - protein, 9 aa, synthetic construct
GGTGVDQLK

SEQ ID NO: 24241 - protein, 9 aa, synthetic construct
GGAGDDRYL

SEQ ID NO: 24242 - protein, 9 aa, synthetic construct
GGTGVDYMD

SEQ ID NO: 24243 - protein, 9 aa, synthetic construct
GGTGVDYMS

SEQ ID NO: 24244 - protein, 9 aa, synthetic construct
GGTGYDTIY

SEQ ID NO: 24245 - protein, 9 aa, synthetic construct
GGAGDDRFL

SEQ ID NO: 24246 - protein, 9 aa, synthetic construct
GGAGDDRFS

SEQ ID NO: 24247 - protein, 9 aa, synthetic construct
GGAGDDRFT

SEQ ID NO: 24248 - protein, 9 aa, synthetic construct
GGVGADFLG

SEQ ID NO: 24249 - protein, 9 aa, synthetic construct
GGVGADFIQ

SEQ ID NO: 24250 - protein, 9 aa, synthetic construct
GGVGADDMQ

SEQ ID NO: 24251 - protein, 9 aa, synthetic construct
GGVGADDLW

SEQ ID NO: 24252 - protein, 9 aa, synthetic construct
GGVGADALT

SEQ ID NO: 24253 - protein, 9 aa, synthetic construct
GGVGADAFI

SEQ ID NO: 24254 - protein, 9 aa, synthetic construct
GGTGYDVMT

SEQ ID NO: 24255 - protein, 9 aa, synthetic construct
GGTGYDTLI

SEQ ID NO: 24256 - protein, 9 aa, synthetic construct
GGTGYDTAS

SEQ ID NO: 24257 - protein, 9 aa, synthetic construct
GGTGWDLAY

SEQ ID NO: 24258 - protein, 9 aa, synthetic construct
GGAGDDRMA

SEQ ID NO: 24259 - protein, 9 aa, synthetic construct
GGAGDDRMF

SEQ ID NO: 24260 - protein, 9 aa, synthetic construct
GGTGYDQLW

SEQ ID NO: 24261 - protein, 9 aa, synthetic construct
GGAGDDRMW

SEQ ID NO: 24262 - protein, 9 aa, synthetic construct
GGTGYDILN

SEQ ID NO: 24263 - protein, 9 aa, synthetic construct
GGAGDDRVL

SEQ ID NO: 24264 - protein, 9 aa, synthetic construct
GGAGDDRVR

SEQ ID NO: 24265 - protein, 9 aa, synthetic construct
GGTGWDWID

SEQ ID NO: 24266 - protein, 9 aa, synthetic construct
GGTGWDVML

SEQ ID NO: 24267 - protein, 9 aa, synthetic construct
GGTGWDVFF

SEQ ID NO: 24268 - protein, 9 aa, synthetic construct
GGAGDDRVS

SEQ ID NO: 24269 - protein, 9 aa, synthetic construct
GGTGSDRLL

SEQ ID NO: 24270 - protein, 9 aa, synthetic construct
GGAGDDVMH

SEQ ID NO: 24271 - protein, 9 aa, synthetic construct
GGAGEDSLR

SEQ ID NO: 24272 - protein, 9 aa, synthetic construct
GGAGEDLLV

SEQ ID NO: 24273 - protein, 9 aa, synthetic construct
GGTGRDHLG

SEQ ID NO: 24274 - protein, 9 aa, synthetic construct
GGTGRDFVS

SEQ ID NO: 24275 - protein, 9 aa, synthetic construct
GGAGEDILL

SEQ ID NO: 24276 - protein, 9 aa, synthetic construct
GGTGRDFLT

SEQ ID NO: 24277 - protein, 9 aa, synthetic construct
GGAGEDILR

SEQ ID NO: 24278 - protein, 9 aa, synthetic construct
GGTGRDELY

SEQ ID NO: 24279 - protein, 9 aa, synthetic construct
GGTGRDELI

SEQ ID NO: 24280 - protein, 9 aa, synthetic construct
GGAGEDIVG

SEQ ID NO: 24281 - protein, 9 aa, synthetic construct
GGEGTDILE

SEQ ID NO: 24282 - protein, 9 aa, synthetic construct
GGTGRDDLS

SEQ ID NO: 24283 - protein, 9 aa, synthetic construct
GGAGEDKLY

SEQ ID NO: 24284 - protein, 9 aa, synthetic construct
GGAGEDLFR

SEQ ID NO: 24285 - protein, 9 aa, synthetic construct
GGAGEDLID

SEQ ID NO: 24286 - protein, 9 aa, synthetic construct
GGAGEDLIF

SEQ ID NO: 24287 - protein, 9 aa, synthetic construct
GGEGNDSIV

SEQ ID NO: 24288 - protein, 9 aa, synthetic construct
GGTGQDYLY

SEQ ID NO: 24289 - protein, 9 aa, synthetic construct
GGAGEDLLE

SEQ ID NO: 24290 - protein, 9 aa, synthetic construct
GGEGTDIMI

SEQ ID NO: 24291 - protein, 9 aa, synthetic construct
GGAGEDLLH

SEQ ID NO: 24292 - protein, 9 aa, synthetic construct
GGTGQDVMY

SEQ ID NO: 24293 - protein, 9 aa, synthetic construct
GGTGQDVMS

SEQ ID NO: 24294 - protein, 9 aa, synthetic construct
GGTGQDVLV

SEQ ID NO: 24295 - protein, 9 aa, synthetic construct
GGAGEDLLL

SEQ ID NO: 24296 - protein, 9 aa, synthetic construct
GGAGEDLLM

SEQ ID NO: 24297 - protein, 9 aa, synthetic construct
GGAGEDLLR

SEQ ID NO: 24298 - protein, 9 aa, synthetic construct
GGTGRDHMF

SEQ ID NO: 24299 - protein, 9 aa, synthetic construct
GGAGEDIFK

SEQ ID NO: 24300 - protein, 9 aa, synthetic construct
GGTGRDIIN

SEQ ID NO: 24301 - protein, 9 aa, synthetic construct
GGEGSDYLY

SEQ ID NO: 24302 - protein, 9 aa, synthetic construct
GGAGEDELF

SEQ ID NO: 24303 - protein, 9 aa, synthetic construct
GGTGRDLMW

SEQ ID NO: 24304 - protein, 9 aa, synthetic construct
GGTGRDLMI

SEQ ID NO: 24305 - protein, 9 aa, synthetic construct
GGTGRDLMA

SEQ ID NO: 24306 - protein, 9 aa, synthetic construct
GGAGEDELT

SEQ ID NO: 24307 - protein, 9 aa, synthetic construct
GGTGRDLLT

SEQ ID NO: 24308 - protein, 9 aa, synthetic construct
GGTGRDLLQ

SEQ ID NO: 24309 - protein, 9 aa, synthetic construct
GGTGRDLLN

SEQ ID NO: 24310 - protein, 9 aa, synthetic construct
GGTGRDLLL

SEQ ID NO: 24311 - protein, 9 aa, synthetic construct
GGAGEDELY

SEQ ID NO: 24312 - protein, 9 aa, synthetic construct
GGTGRDLLA

SEQ ID NO: 24313 - protein, 9 aa, synthetic construct
GGAGEDFIM

SEQ ID NO: 24314 - protein, 9 aa, synthetic construct
GGTGRDILL

SEQ ID NO: 24315 - protein, 9 aa, synthetic construct
GGEGSDYMN

SEQ ID NO: 24316 - protein, 9 aa, synthetic construct
GGTGRDKVF

SEQ ID NO: 24317 - protein, 9 aa, synthetic construct
GGAGEDGFG

SEQ ID NO: 24318 - protein, 9 aa, synthetic construct
GGTGRDKLI

SEQ ID NO: 24319 - protein, 9 aa, synthetic construct
GGTGRDKFV

SEQ ID NO: 24320 - protein, 9 aa, synthetic construct
GGEGTDFLF

SEQ ID NO: 24321 - protein, 9 aa, synthetic construct
GGTGRDIVY

SEQ ID NO: 24322 - protein, 9 aa, synthetic construct
GGEGTDFLY

SEQ ID NO: 24323 - protein, 9 aa, synthetic construct
GGEGTDGLH

SEQ ID NO: 24324 - protein, 9 aa, synthetic construct
GGAGEDHLE

SEQ ID NO: 24325 - protein, 9 aa, synthetic construct
GGTGRDIMS

SEQ ID NO: 24326 - protein, 9 aa, synthetic construct
GGAGEDLLS

SEQ ID NO: 24327 - protein, 9 aa, synthetic construct
GGTGQDVLF

SEQ ID NO: 24328 - protein, 9 aa, synthetic construct
GGEGNDSMS

SEQ ID NO: 24329 - protein, 9 aa, synthetic construct
GGAGEDLVR

SEQ ID NO: 24330 - protein, 9 aa, synthetic construct
GGTGQDMIA

SEQ ID NO: 24331 - protein, 9 aa, synthetic construct
GGEGNDSFR

SEQ ID NO: 24332 - protein, 9 aa, synthetic construct
GGAGEDRFL

SEQ ID NO: 24333 - protein, 9 aa, synthetic construct
GGTGQDLLT

SEQ ID NO: 24334 - protein, 9 aa, synthetic construct
GGEGNDSFE

SEQ ID NO: 24335 - protein, 9 aa, synthetic construct
GGEGTDRAS

SEQ ID NO: 24336 - protein, 9 aa, synthetic construct
GGAGEDRIE

SEQ ID NO: 24337 - protein, 9 aa, synthetic construct
GGTGQDKLY

SEQ ID NO: 24338 - protein, 9 aa, synthetic construct
GGTGQDILT

SEQ ID NO: 24339 - protein, 9 aa, synthetic construct
GGAGEDRIS

SEQ ID NO: 24340 - protein, 9 aa, synthetic construct
GGTGQDILN

SEQ ID NO: 24341 - protein, 9 aa, synthetic construct
GGTGQDILE

SEQ ID NO: 24342 - protein, 9 aa, synthetic construct
GGAGEDRLA

SEQ ID NO: 24343 - protein, 9 aa, synthetic construct
GGAGEDRLM

SEQ ID NO: 24344 - protein, 9 aa, synthetic construct
GGTGQDFLQ

SEQ ID NO: 24345 - protein, 9 aa, synthetic construct
GGAGEDRLT

SEQ ID NO: 24346 - protein, 9 aa, synthetic construct
GGAGEDRLV

SEQ ID NO: 24347 - protein, 9 aa, synthetic construct
GGTGPDTMT

SEQ ID NO: 24348 - protein, 9 aa, synthetic construct
GGAGEDRVV

SEQ ID NO: 24349 - protein, 9 aa, synthetic construct
GGEGTDSLL

SEQ ID NO: 24350 - protein, 9 aa, synthetic construct
GGTGPDSLT

SEQ ID NO: 24351 - protein, 9 aa, synthetic construct
GGTGPDQMI

SEQ ID NO: 24352 - protein, 9 aa, synthetic construct
GGTGPDQLF

SEQ ID NO: 24353 - protein, 9 aa, synthetic construct
GGTGPDMLI

SEQ ID NO: 24354 - protein, 9 aa, synthetic construct
GGEGTDSVD

SEQ ID NO: 24355 - protein, 9 aa, synthetic construct
GGAGEDQLY

SEQ ID NO: 24356 - protein, 9 aa, synthetic construct
GGAGEDQLW

SEQ ID NO: 24357 - protein, 9 aa, synthetic construct
GGAGEDQLF

SEQ ID NO: 24358 - protein, 9 aa, synthetic construct
GGTGQDTIA

SEQ ID NO: 24359 - protein, 9 aa, synthetic construct
GGEGNDSIT

SEQ ID NO: 24360 - protein, 9 aa, synthetic construct
GGTGQDTVL

SEQ ID NO: 24361 - protein, 9 aa, synthetic construct
GGAGEDLYV

SEQ ID NO: 24362 - protein, 9 aa, synthetic construct
GGTGQDTMV

SEQ ID NO: 24363 - protein, 9 aa, synthetic construct
GGEGTDIYI

SEQ ID NO: 24364 - protein, 9 aa, synthetic construct
GGAGEDMAI

SEQ ID NO: 24365 - protein, 9 aa, synthetic construct
GGEGTDKAV

SEQ ID NO: 24366 - protein, 9 aa, synthetic construct
GGTGQDTLL

SEQ ID NO: 24367 - protein, 9 aa, synthetic construct
GGAGEDMLN

SEQ ID NO: 24368 - protein, 9 aa, synthetic construct
GGTGQDTIN

SEQ ID NO: 24369 - protein, 9 aa, synthetic construct
GGEGNDSIN

SEQ ID NO: 24370 - protein, 9 aa, synthetic construct
GGEGTDKLY

SEQ ID NO: 24371 - protein, 9 aa, synthetic construct
GGTGQDQLR

SEQ ID NO: 24372 - protein, 9 aa, synthetic construct
GGEGNDSIK

SEQ ID NO: 24373 - protein, 9 aa, synthetic construct
GGTGQDSLS

SEQ ID NO: 24374 - protein, 9 aa, synthetic construct
GGTGQDSIL

SEQ ID NO: 24375 - protein, 9 aa, synthetic construct
GGEGTDLAS

SEQ ID NO: 24376 - protein, 9 aa, synthetic construct
GGAGEDNLQ

SEQ ID NO: 24377 - protein, 9 aa, synthetic construct
GGTGQDRLS

SEQ ID NO: 24378 - protein, 9 aa, synthetic construct
GGTGQDRLL

SEQ ID NO: 24379 - protein, 9 aa, synthetic construct
GGAGEDQIE

SEQ ID NO: 24380 - protein, 9 aa, synthetic construct
GGEGNDSIE

SEQ ID NO: 24381 - protein, 9 aa, synthetic construct
GGAGEDQLA

SEQ ID NO: 24382 - protein, 9 aa, synthetic construct
GGAGEDQLD

SEQ ID NO: 24383 - protein, 9 aa, synthetic construct
GGEGSDYLD

SEQ ID NO: 24384 - protein, 9 aa, synthetic construct
GGTGRDMLY

SEQ ID NO: 24385 - protein, 9 aa, synthetic construct
GGTGSDQLL

SEQ ID NO: 24386 - protein, 9 aa, synthetic construct
GGTGSDALH

SEQ ID NO: 24387 - protein, 9 aa, synthetic construct
GGTGSDIIV

SEQ ID NO: 24388 - protein, 9 aa, synthetic construct
GGTGSDIFL

SEQ ID NO: 24389 - protein, 9 aa, synthetic construct
GGEGNDTAT

SEQ ID NO: 24390 - protein, 9 aa, synthetic construct
GGEGNDTAS

SEQ ID NO: 24391 - protein, 9 aa, synthetic construct
GGTGSDHLT

SEQ ID NO: 24392 - protein, 9 aa, synthetic construct
GGEGSDVIN

SEQ ID NO: 24393 - protein, 9 aa, synthetic construct
GGTGSDHIF

SEQ ID NO: 24394 - protein, 9 aa, synthetic construct
GGEGSDVIT

SEQ ID NO: 24395 - protein, 9 aa, synthetic construct
GGTGSDFID

SEQ ID NO: 24396 - protein, 9 aa, synthetic construct
GGTGSDELY

SEQ ID NO: 24397 - protein, 9 aa, synthetic construct
GGTGSDELS

SEQ ID NO: 24398 - protein, 9 aa, synthetic construct
GGEGNDTAR

SEQ ID NO: 24399 - protein, 9 aa, synthetic construct
GGEGSDVLA

SEQ ID NO: 24400 - protein, 9 aa, synthetic construct
GGTGSDEAH

SEQ ID NO: 24401 - protein, 9 aa, synthetic construct
GGTGSDDMT

SEQ ID NO: 24402 - protein, 9 aa, synthetic construct
GGEGSDVLE

SEQ ID NO: 24403 - protein, 9 aa, synthetic construct
GGEGSDVLI

SEQ ID NO: 24404 - protein, 9 aa, synthetic construct
GGTGSDDLR

SEQ ID NO: 24405 - protein, 9 aa, synthetic construct
GGTGSDDLI

SEQ ID NO: 24406 - protein, 9 aa, synthetic construct
GGEGSDVLL

SEQ ID NO: 24407 - protein, 9 aa, synthetic construct
GGEGSDVLN

SEQ ID NO: 24408 - protein, 9 aa, synthetic construct
GGEGSDVLS

SEQ ID NO: 24409 - protein, 9 aa, synthetic construct
GGTGSDAYV

SEQ ID NO: 24410 - protein, 9 aa, synthetic construct
GGTGSDAMT

SEQ ID NO: 24411 - protein, 9 aa, synthetic construct
GGTGSDAMR

SEQ ID NO: 24412 - protein, 9 aa, synthetic construct
GGAGDDWIH

SEQ ID NO: 24413 - protein, 9 aa, synthetic construct
GGAGDDWIG

SEQ ID NO: 24414 - protein, 9 aa, synthetic construct
GGTGSDILF

SEQ ID NO: 24415 - protein, 9 aa, synthetic construct
GGTGSDLLL

SEQ ID NO: 24416 - protein, 9 aa, synthetic construct
GGTGSDQLH

SEQ ID NO: 24417 - protein, 9 aa, synthetic construct
GGTGSDQLA

SEQ ID NO: 24418 - protein, 9 aa, synthetic construct
GGTGSDNAY

SEQ ID NO: 24419 - protein, 9 aa, synthetic construct
GGTGSDMLN

SEQ ID NO: 24420 - protein, 9 aa, synthetic construct
GGTGSDMLD

SEQ ID NO: 24421 - protein, 9 aa, synthetic construct
GGTGSDMLA

SEQ ID NO: 24422 - protein, 9 aa, synthetic construct
GGEGSDVFG

SEQ ID NO: 24423 - protein, 9 aa, synthetic construct
GGTGSDLYL

SEQ ID NO: 24424 - protein, 9 aa, synthetic construct
GGTGSDLMT

SEQ ID NO: 24425 - protein, 9 aa, synthetic construct
GGTGSDLLR

SEQ ID NO: 24426 - protein, 9 aa, synthetic construct
GGTGSDLLN

SEQ ID NO: 24427 - protein, 9 aa, synthetic construct
GGTGSDLLI

SEQ ID NO: 24428 - protein, 9 aa, synthetic construct
GGAGDDWFS

SEQ ID NO: 24429 - protein, 9 aa, synthetic construct
GGTGSDLLE

SEQ ID NO: 24430 - protein, 9 aa, synthetic construct
GGTGSDLLA

SEQ ID NO: 24431 - protein, 9 aa, synthetic construct
GGTGSDLIT

SEQ ID NO: 24432 - protein, 9 aa, synthetic construct
GGTGSDLFV

SEQ ID NO: 24433 - protein, 9 aa, synthetic construct
GGAGDDVYN

SEQ ID NO: 24434 - protein, 9 aa, synthetic construct
GGTGSDKLT

SEQ ID NO: 24435 - protein, 9 aa, synthetic construct
GGTGSDKLI

SEQ ID NO: 24436 - protein, 9 aa, synthetic construct
GGTGSDKLF

SEQ ID NO: 24437 - protein, 9 aa, synthetic construct
GGEGSDVFN

SEQ ID NO: 24438 - protein, 9 aa, synthetic construct
GGTGSDIYQ

SEQ ID NO: 24439 - protein, 9 aa, synthetic construct
GGEGSDVFR

SEQ ID NO: 24440 - protein, 9 aa, synthetic construct
GGTGSDALN

SEQ ID NO: 24441 - protein, 9 aa, synthetic construct
GGEGNDTAF

SEQ ID NO: 24442 - protein, 9 aa, synthetic construct
GGAGEDEFV

SEQ ID NO: 24443 - protein, 9 aa, synthetic construct
GGEGNDTAD

SEQ ID NO: 24444 - protein, 9 aa, synthetic construct
GGAGDDYMM

SEQ ID NO: 24445 - protein, 9 aa, synthetic construct
GGTGRDTIL

SEQ ID NO: 24446 - protein, 9 aa, synthetic construct
GGAGDDYVH

SEQ ID NO: 24447 - protein, 9 aa, synthetic construct
GGAGDDYVR

SEQ ID NO: 24448 - protein, 9 aa, synthetic construct
GGAGDDYVT

SEQ ID NO: 24449 - protein, 9 aa, synthetic construct
GGEGSDVYV

SEQ ID NO: 24450 - protein, 9 aa, synthetic construct
GGEGNDSVV

SEQ ID NO: 24451 - protein, 9 aa, synthetic construct
GGTGRDSLT

SEQ ID NO: 24452 - protein, 9 aa, synthetic construct
GGTGRDSLR

SEQ ID NO: 24453 - protein, 9 aa, synthetic construct
GGTGRDSLL

SEQ ID NO: 24454 - protein, 9 aa, synthetic construct
GGTGRDSLI

SEQ ID NO: 24455 - protein, 9 aa, synthetic construct
GGAGEDAIS

SEQ ID NO: 24456 - protein, 9 aa, synthetic construct
GGTGRDRVL

SEQ ID NO: 24457 - protein, 9 aa, synthetic construct
GGEGNDSVM

SEQ ID NO: 24458 - protein, 9 aa, synthetic construct
GGEGSDWIE

SEQ ID NO: 24459 - protein, 9 aa, synthetic construct
GGTGRDRLT

SEQ ID NO: 24460 - protein, 9 aa, synthetic construct
GGEGNDSVL

SEQ ID NO: 24461 - protein, 9 aa, synthetic construct
GGTGRDRIF

SEQ ID NO: 24462 - protein, 9 aa, synthetic construct
GGTGRDRAF

SEQ ID NO: 24463 - protein, 9 aa, synthetic construct
GGTGRDQVD

SEQ ID NO: 24464 - protein, 9 aa, synthetic construct
GGAGEDDLA

SEQ ID NO: 24465 - protein, 9 aa, synthetic construct
GGTGRDQLF

SEQ ID NO: 24466 - protein, 9 aa, synthetic construct
GGAGEDDLG

SEQ ID NO: 24467 - protein, 9 aa, synthetic construct
GGAGEDDMD

SEQ ID NO: 24468 - protein, 9 aa, synthetic construct
GGEGSDYID

SEQ ID NO: 24469 - protein, 9 aa, synthetic construct
GGTGRDTIS

SEQ ID NO: 24470 - protein, 9 aa, synthetic construct
GGTGRDTLQ

SEQ ID NO: 24471 - protein, 9 aa, synthetic construct
GGTGRDTLY

SEQ ID NO: 24472 - protein, 9 aa, synthetic construct
GGTGRDVMT

SEQ ID NO: 24473 - protein, 9 aa, synthetic construct
GGTGSDAFV

SEQ ID NO: 24474 - protein, 9 aa, synthetic construct
GGTGSDAAS

SEQ ID NO: 24475 - protein, 9 aa, synthetic construct
GGAGDDYFY

SEQ ID NO: 24476 - protein, 9 aa, synthetic construct
GGTGRDYLV

SEQ ID NO: 24477 - protein, 9 aa, synthetic construct
GGTGRDYLS

SEQ ID NO: 24478 - protein, 9 aa, synthetic construct
GGTGRDYIE

SEQ ID NO: 24479 - protein, 9 aa, synthetic construct
GGEGNDTAA

SEQ ID NO: 24480 - protein, 9 aa, synthetic construct
GGTGRDWLV

SEQ ID NO: 24481 - protein, 9 aa, synthetic construct
GGTGRDWLI

SEQ ID NO: 24482 - protein, 9 aa, synthetic construct
GGTGRDWLA

SEQ ID NO: 24483 - protein, 9 aa, synthetic construct
GGAGDDYIY

SEQ ID NO: 24484 - protein, 9 aa, synthetic construct
GGTGRDVLR

SEQ ID NO: 24485 - protein, 9 aa, synthetic construct
GGTGRDTML

SEQ ID NO: 24486 - protein, 9 aa, synthetic construct
GGTGRDVLK

SEQ ID NO: 24487 - protein, 9 aa, synthetic construct
GGTGRDVLA

SEQ ID NO: 24488 - protein, 9 aa, synthetic construct
GGTGRDVIQ

SEQ ID NO: 24489 - protein, 9 aa, synthetic construct
GGAGDDYLM

SEQ ID NO: 24490 - protein, 9 aa, synthetic construct
GGTGRDVIA

SEQ ID NO: 24491 - protein, 9 aa, synthetic construct
GGTGRDVFR

SEQ ID NO: 24492 - protein, 9 aa, synthetic construct
GGTGRDVFL

SEQ ID NO: 24493 - protein, 9 aa, synthetic construct
GGTGRDVAA

SEQ ID NO: 24494 - protein, 9 aa, synthetic construct
GGTGRDTVS

SEQ ID NO: 24495 - protein, 9 aa, synthetic construct
GGTGRDTMR

SEQ ID NO: 24496 - protein, 9 aa, synthetic construct
GGAGDDYMD

SEQ ID NO: 24497 - protein, 9 aa, synthetic construct
GGSGADMIS

SEQ ID NO: 24498 - protein, 9 aa, synthetic construct
GGAGNDNVF

SEQ ID NO: 24499 - protein, 9 aa, synthetic construct
GGSGADLYL

SEQ ID NO: 24500 - protein, 9 aa, synthetic construct
GGAGYDDLR

SEQ ID NO: 24501 - protein, 9 aa, synthetic construct
GGPGDDIYF

SEQ ID NO: 24502 - protein, 9 aa, synthetic construct
GGGGDDSVR

SEQ ID NO: 24503 - protein, 9 aa, synthetic construct
GGAGYDMMS

SEQ ID NO: 24504 - protein, 9 aa, synthetic construct
GGEGEDIIE

SEQ ID NO: 24505 - protein, 9 aa, synthetic construct
GGPGDDIMF

SEQ ID NO: 24506 - protein, 9 aa, synthetic construct
GGAGYDNLT

SEQ ID NO: 24507 - protein, 9 aa, synthetic construct
GGAGYDQIH

SEQ ID NO: 24508 - protein, 9 aa, synthetic construct
GGPGDDILT

SEQ ID NO: 24509 - protein, 9 aa, synthetic construct
GGPGDDILE

SEQ ID NO: 24510 - protein, 9 aa, synthetic construct
GGPGDDILD

SEQ ID NO: 24511 - protein, 9 aa, synthetic construct
GGPGDDILA

SEQ ID NO: 24512 - protein, 9 aa, synthetic construct
GGPGDDIIV

SEQ ID NO: 24513 - protein, 9 aa, synthetic construct
GGGGDDTAT

SEQ ID NO: 24514 - protein, 9 aa, synthetic construct
GGPGDDIID

SEQ ID NO: 24515 - protein, 9 aa, synthetic construct
GGPGDDIFV

SEQ ID NO: 24516 - protein, 9 aa, synthetic construct
GGAGYDQLN

SEQ ID NO: 24517 - protein, 9 aa, synthetic construct
GGEGEDIFK

SEQ ID NO: 24518 - protein, 9 aa, synthetic construct
GGGGDDTAW

SEQ ID NO: 24519 - protein, 9 aa, synthetic construct
GGGGDDTFD

SEQ ID NO: 24520 - protein, 9 aa, synthetic construct
GGPGDDHLI

SEQ ID NO: 24521 - protein, 9 aa, synthetic construct
GGEGEDIAL

SEQ ID NO: 24522 - protein, 9 aa, synthetic construct
GGPGDDHLA

SEQ ID NO: 24523 - protein, 9 aa, synthetic construct
GGPGDDGVI

SEQ ID NO: 24524 - protein, 9 aa, synthetic construct
GGPGDDGLY

SEQ ID NO: 24525 - protein, 9 aa, synthetic construct
GGAGYDRLI

SEQ ID NO: 24526 - protein, 9 aa, synthetic construct
GGPGDDIYN

SEQ ID NO: 24527 - protein, 9 aa, synthetic construct
GGAGYDMLI

SEQ ID NO: 24528 - protein, 9 aa, synthetic construct
GGPGDDIYY

SEQ ID NO: 24529 - protein, 9 aa, synthetic construct
GGPGDDLVI

SEQ ID NO: 24530 - protein, 9 aa, synthetic construct
GGPGDDQLH

SEQ ID NO: 24531 - protein, 9 aa, synthetic construct
GGAGYDELQ

SEQ ID NO: 24532 - protein, 9 aa, synthetic construct
GGAGYDFIA

SEQ ID NO: 24533 - protein, 9 aa, synthetic construct
GGPGDDNLS

SEQ ID NO: 24534 - protein, 9 aa, synthetic construct
GGPGDDNLM

SEQ ID NO: 24535 - protein, 9 aa, synthetic construct
GGPGDDNLD

SEQ ID NO: 24536 - protein, 9 aa, synthetic construct
GGGGDDSLK

SEQ ID NO: 24537 - protein, 9 aa, synthetic construct
GGPGDDMMD

SEQ ID NO: 24538 - protein, 9 aa, synthetic construct
GGPGDDMLT

SEQ ID NO: 24539 - protein, 9 aa, synthetic construct
GGAGYDIFD

SEQ ID NO: 24540 - protein, 9 aa, synthetic construct
GGAGYDILI

SEQ ID NO: 24541 - protein, 9 aa, synthetic construct
GGPGDDLMQ

SEQ ID NO: 24542 - protein, 9 aa, synthetic construct
GGAGYDMLD

SEQ ID NO: 24543 - protein, 9 aa, synthetic construct
GGAGYDKAL

SEQ ID NO: 24544 - protein, 9 aa, synthetic construct
GGPGDDLIY

SEQ ID NO: 24545 - protein, 9 aa, synthetic construct
GGAGYDLLD

SEQ ID NO: 24546 - protein, 9 aa, synthetic construct
GGPGDDLIT

SEQ ID NO: 24547 - protein, 9 aa, synthetic construct
GGEGEDILT

SEQ ID NO: 24548 - protein, 9 aa, synthetic construct
GGAGYDLLS

SEQ ID NO: 24549 - protein, 9 aa, synthetic construct
GGAGYDLLT

SEQ ID NO: 24550 - protein, 9 aa, synthetic construct
GGEGEDILI

SEQ ID NO: 24551 - protein, 9 aa, synthetic construct
GGPGDDLFI

SEQ ID NO: 24552 - protein, 9 aa, synthetic construct
GGPGDDKLW

SEQ ID NO: 24553 - protein, 9 aa, synthetic construct
GGAGYDLVL

SEQ ID NO: 24554 - protein, 9 aa, synthetic construct
GGAGYDRLT

SEQ ID NO: 24555 - protein, 9 aa, synthetic construct
GGAGYDRLV

SEQ ID NO: 24556 - protein, 9 aa, synthetic construct
GGPGDDFLV

SEQ ID NO: 24557 - protein, 9 aa, synthetic construct
GGAGYDYYI

SEQ ID NO: 24558 - protein, 9 aa, synthetic construct
GGAGYDWIY

SEQ ID NO: 24559 - protein, 9 aa, synthetic construct
GGPGADVLE

SEQ ID NO: 24560 - protein, 9 aa, synthetic construct
GGAGYDWLF

SEQ ID NO: 24561 - protein, 9 aa, synthetic construct
GGPGADVIR

SEQ ID NO: 24562 - protein, 9 aa, synthetic construct
GGPGADVFR

SEQ ID NO: 24563 - protein, 9 aa, synthetic construct
GGPGADVFI

SEQ ID NO: 24564 - protein, 9 aa, synthetic construct
GGPGADVFA

SEQ ID NO: 24565 - protein, 9 aa, synthetic construct
GGPGADTYV

SEQ ID NO: 24566 - protein, 9 aa, synthetic construct
GGPGADTYL

SEQ ID NO: 24567 - protein, 9 aa, synthetic construct
GGPGADTVY

SEQ ID NO: 24568 - protein, 9 aa, synthetic construct
GGPGADTMR

SEQ ID NO: 24569 - protein, 9 aa, synthetic construct
GGCGADTIY

SEQ ID NO: 24570 - protein, 9 aa, synthetic construct
GGAGYDVLV

SEQ ID NO: 24571 - protein, 9 aa, synthetic construct
GGGGDDTMQ

SEQ ID NO: 24572 - protein, 9 aa, synthetic construct
GGPGADTIA

SEQ ID NO: 24573 - protein, 9 aa, synthetic construct
GGPGADTFM

SEQ ID NO: 24574 - protein, 9 aa, synthetic construct
GGPGADTFI

SEQ ID NO: 24575 - protein, 9 aa, synthetic construct
GGPGADSLT

SEQ ID NO: 24576 - protein, 9 aa, synthetic construct
GGCGDDTLV

SEQ ID NO: 24577 - protein, 9 aa, synthetic construct
GGPGADSLN

SEQ ID NO: 24578 - protein, 9 aa, synthetic construct
GGCGDDVLH

SEQ ID NO: 24579 - protein, 9 aa, synthetic construct
GGPGADSLD

SEQ ID NO: 24580 - protein, 9 aa, synthetic construct
GGPGADSID

SEQ ID NO: 24581 - protein, 9 aa, synthetic construct
GGPGADSFV

SEQ ID NO: 24582 - protein, 9 aa, synthetic construct
GGPGADVLQ

SEQ ID NO: 24583 - protein, 9 aa, synthetic construct
GGGGDDTLG

SEQ ID NO: 24584 - protein, 9 aa, synthetic construct
GGPGDDFLT

SEQ ID NO: 24585 - protein, 9 aa, synthetic construct
GGEGEDFLY

SEQ ID NO: 24586 - protein, 9 aa, synthetic construct
GGPGDDFLS

SEQ ID NO: 24587 - protein, 9 aa, synthetic construct
GGPGDDFLR

SEQ ID NO: 24588 - protein, 9 aa, synthetic construct
GGPGDDFLN

SEQ ID NO: 24589 - protein, 9 aa, synthetic construct
GGAGYDRMM

SEQ ID NO: 24590 - protein, 9 aa, synthetic construct
GGPGDDELY

SEQ ID NO: 24591 - protein, 9 aa, synthetic construct
GGPGDDELR

SEQ ID NO: 24592 - protein, 9 aa, synthetic construct
GGPGDDEIH

SEQ ID NO: 24593 - protein, 9 aa, synthetic construct
GGGGDDTIG

SEQ ID NO: 24594 - protein, 9 aa, synthetic construct
GGPGDDDLS

SEQ ID NO: 24595 - protein, 9 aa, synthetic construct
GGPGDDDLR

SEQ ID NO: 24596 - protein, 9 aa, synthetic construct
GGPGDDDLN

SEQ ID NO: 24597 - protein, 9 aa, synthetic construct
GGAGYDTFY

SEQ ID NO: 24598 - protein, 9 aa, synthetic construct
GGAGYDVFQ

SEQ ID NO: 24599 - protein, 9 aa, synthetic construct
GGAGYDTIR

SEQ ID NO: 24600 - protein, 9 aa, synthetic construct
GGGGDDTIM

SEQ ID NO: 24601 - protein, 9 aa, synthetic construct
GGPGDDALD

SEQ ID NO: 24602 - protein, 9 aa, synthetic construct
GGGGDDTIQ

SEQ ID NO: 24603 - protein, 9 aa, synthetic construct
GGPGDDAIT

SEQ ID NO: 24604 - protein, 9 aa, synthetic construct
GGEGEDFLT

SEQ ID NO: 24605 - protein, 9 aa, synthetic construct
GGPGCDTLL

SEQ ID NO: 24606 - protein, 9 aa, synthetic construct
GGAGYDTLY

SEQ ID NO: 24607 - protein, 9 aa, synthetic construct
GGPGADYFI

SEQ ID NO: 24608 - protein, 9 aa, synthetic construct
GGPGADWLM

SEQ ID NO: 24609 - protein, 9 aa, synthetic construct
GGPGADWLL

SEQ ID NO: 24610 - protein, 9 aa, synthetic construct
GGPGDDQLL

SEQ ID NO: 24611 - protein, 9 aa, synthetic construct
GGPGDDRIK

SEQ ID NO: 24612 - protein, 9 aa, synthetic construct
GGPGHDRIL

SEQ ID NO: 24613 - protein, 9 aa, synthetic construct
GGPGDDRIM

SEQ ID NO: 24614 - protein, 9 aa, synthetic construct
GGAGVDVFR

SEQ ID NO: 24615 - protein, 9 aa, synthetic construct
GGAGVDVFV

SEQ ID NO: 24616 - protein, 9 aa, synthetic construct
GGAGVDVIS

SEQ ID NO: 24617 - protein, 9 aa, synthetic construct
GGPGFDTLD

SEQ ID NO: 24618 - protein, 9 aa, synthetic construct
GGAGVDVIT

SEQ ID NO: 24619 - protein, 9 aa, synthetic construct
GGPGFDRLI

SEQ ID NO: 24620 - protein, 9 aa, synthetic construct
GGGGDDQMT

SEQ ID NO: 24621 - protein, 9 aa, synthetic construct
GGAGVDVLQ

SEQ ID NO: 24622 - protein, 9 aa, synthetic construct
GGAGVDVLR

SEQ ID NO: 24623 - protein, 9 aa, synthetic construct
GGAGVDVLY

SEQ ID NO: 24624 - protein, 9 aa, synthetic construct
GGPGFDELI

SEQ ID NO: 24625 - protein, 9 aa, synthetic construct
GGAGVDVMD

SEQ ID NO: 24626 - protein, 9 aa, synthetic construct
GGAGVDVMT

SEQ ID NO: 24627 - protein, 9 aa, synthetic construct
GGGGDDQVS

SEQ ID NO: 24628 - protein, 9 aa, synthetic construct
GGPGEDVIS

SEQ ID NO: 24629 - protein, 9 aa, synthetic construct
GGEGEDRLF

SEQ ID NO: 24630 - protein, 9 aa, synthetic construct
GGEGEDRLE

SEQ ID NO: 24631 - protein, 9 aa, synthetic construct
GGPGEDTMR

SEQ ID NO: 24632 - protein, 9 aa, synthetic construct
GGAGVDWVD

SEQ ID NO: 24633 - protein, 9 aa, synthetic construct
GGAGVDYAT

SEQ ID NO: 24634 - protein, 9 aa, synthetic construct
GGPGEDSLY

SEQ ID NO: 24635 - protein, 9 aa, synthetic construct
GGPGEDSLF

SEQ ID NO: 24636 - protein, 9 aa, synthetic construct
GGGGDDRIA

SEQ ID NO: 24637 - protein, 9 aa, synthetic construct
GGAGVDYLA

SEQ ID NO: 24638 - protein, 9 aa, synthetic construct
GGAGVDYLT

SEQ ID NO: 24639 - protein, 9 aa, synthetic construct
GGAGVDVFL

SEQ ID NO: 24640 - protein, 9 aa, synthetic construct
GGPGFDVFV

SEQ ID NO: 24641 - protein, 9 aa, synthetic construct
GGGGDDQML

SEQ ID NO: 24642 - protein, 9 aa, synthetic construct
GGPGGDVFV

SEQ ID NO: 24643 - protein, 9 aa, synthetic construct
GGPGHDMLM

SEQ ID NO: 24644 - protein, 9 aa, synthetic construct
GGPGHDMLI

SEQ ID NO: 24645 - protein, 9 aa, synthetic construct
GGPGHDLLL

SEQ ID NO: 24646 - protein, 9 aa, synthetic construct
GGAGVDTLG

SEQ ID NO: 24647 - protein, 9 aa, synthetic construct
GGAGVDTLH

SEQ ID NO: 24648 - protein, 9 aa, synthetic construct
GGPGHDHLN

SEQ ID NO: 24649 - protein, 9 aa, synthetic construct
GGPGHDDLL

SEQ ID NO: 24650 - protein, 9 aa, synthetic construct
GGEGEDSIN

SEQ ID NO: 24651 - protein, 9 aa, synthetic construct
GGPGGDVVQ

SEQ ID NO: 24652 - protein, 9 aa, synthetic construct
GGPGGDVLN

SEQ ID NO: 24653 - protein, 9 aa, synthetic construct
GGPGGDVLD

SEQ ID NO: 24654 - protein, 9 aa, synthetic construct
GGGGDDQLN

SEQ ID NO: 24655 - protein, 9 aa, synthetic construct
GGAGVDVFA

SEQ ID NO: 24656 - protein, 9 aa, synthetic construct
GGAGVDTMM

SEQ ID NO: 24657 - protein, 9 aa, synthetic construct
GGAGVDTMR

SEQ ID NO: 24658 - protein, 9 aa, synthetic construct
GGPGGDTFV

SEQ ID NO: 24659 - protein, 9 aa, synthetic construct
GGPGGDRLL

SEQ ID NO: 24660 - protein, 9 aa, synthetic construct
GGAGVDTVA

SEQ ID NO: 24661 - protein, 9 aa, synthetic construct
GGPGGDRLD

SEQ ID NO: 24662 - protein, 9 aa, synthetic construct
GGPGGDQFA

SEQ ID NO: 24663 - protein, 9 aa, synthetic construct
GGAGVDTVK

SEQ ID NO: 24664 - protein, 9 aa, synthetic construct
GGPGGDIMY

SEQ ID NO: 24665 - protein, 9 aa, synthetic construct
GGPGGDIFC

SEQ ID NO: 24666 - protein, 9 aa, synthetic construct
GGPGFDVLF

SEQ ID NO: 24667 - protein, 9 aa, synthetic construct
GGPGEDHVD

SEQ ID NO: 24668 - protein, 9 aa, synthetic construct
GGPGEDALF

SEQ ID NO: 24669 - protein, 9 aa, synthetic construct
GGAGVDYVE

SEQ ID NO: 24670 - protein, 9 aa, synthetic construct
GGPGDDSLV

SEQ ID NO: 24671 - protein, 9 aa, synthetic construct
GGPGDDTIT

SEQ ID NO: 24672 - protein, 9 aa, synthetic construct
GGAGWDTLI

SEQ ID NO: 24673 - protein, 9 aa, synthetic construct
GGPGDDTIH

SEQ ID NO: 24674 - protein, 9 aa, synthetic construct
GGEGEDLLN

SEQ ID NO: 24675 - protein, 9 aa, synthetic construct
GGPGDDTIF

SEQ ID NO: 24676 - protein, 9 aa, synthetic construct
GGPGDDTIE

SEQ ID NO: 24677 - protein, 9 aa, synthetic construct
GGGGDDRMY

SEQ ID NO: 24678 - protein, 9 aa, synthetic construct
GGEGEDLLL

SEQ ID NO: 24679 - protein, 9 aa, synthetic construct
GGEGEDLLD

SEQ ID NO: 24680 - protein, 9 aa, synthetic construct
GGEGEDLIY

SEQ ID NO: 24681 - protein, 9 aa, synthetic construct
GGPGDDSMS

SEQ ID NO: 24682 - protein, 9 aa, synthetic construct
GGPGDDSLR

SEQ ID NO: 24683 - protein, 9 aa, synthetic construct
GGPGDDTLG

SEQ ID NO: 24684 - protein, 9 aa, synthetic construct
GGPGDDSLF

SEQ ID NO: 24685 - protein, 9 aa, synthetic construct
GGPGDDSLA

SEQ ID NO: 24686 - protein, 9 aa, synthetic construct
GGAGWDVFV

SEQ ID NO: 24687 - protein, 9 aa, synthetic construct
GGPGDDSIS

SEQ ID NO: 24688 - protein, 9 aa, synthetic construct
GGGGDDSIG

SEQ ID NO: 24689 - protein, 9 aa, synthetic construct
GGPGDDSIF

SEQ ID NO: 24690 - protein, 9 aa, synthetic construct
GGAGWDVLN

SEQ ID NO: 24691 - protein, 9 aa, synthetic construct
GGEGEDLIT

SEQ ID NO: 24692 - protein, 9 aa, synthetic construct
GGPGDDRLV

SEQ ID NO: 24693 - protein, 9 aa, synthetic construct
GGPGDDRLI

SEQ ID NO: 24694 - protein, 9 aa, synthetic construct
GGAGYDAAS

SEQ ID NO: 24695 - protein, 9 aa, synthetic construct
GGPGDDTLC

SEQ ID NO: 24696 - protein, 9 aa, synthetic construct
GGPGDDTLM

SEQ ID NO: 24697 - protein, 9 aa, synthetic construct
GGAGWDEAV

SEQ ID NO: 24698 - protein, 9 aa, synthetic construct
GGEGEDNLD

SEQ ID NO: 24699 - protein, 9 aa, synthetic construct
GGPGDDYLS

SEQ ID NO: 24700 - protein, 9 aa, synthetic construct
GGGGDDRIN

SEQ ID NO: 24701 - protein, 9 aa, synthetic construct
GGPGDDWLR

SEQ ID NO: 24702 - protein, 9 aa, synthetic construct
GGPGDDWLF

SEQ ID NO: 24703 - protein, 9 aa, synthetic construct
GGPGDDWLA

SEQ ID NO: 24704 - protein, 9 aa, synthetic construct
GGPGDDWID

SEQ ID NO: 24705 - protein, 9 aa, synthetic construct
GGPGDDWFN

SEQ ID NO: 24706 - protein, 9 aa, synthetic construct
GGPGDDVYL

SEQ ID NO: 24707 - protein, 9 aa, synthetic construct
GGAGWDLAT

SEQ ID NO: 24708 - protein, 9 aa, synthetic construct
GGPGDDVVR

SEQ ID NO: 24709 - protein, 9 aa, synthetic construct
GGPGDDVVG

SEQ ID NO: 24710 - protein, 9 aa, synthetic construct
GGPGDDVMT

SEQ ID NO: 24711 - protein, 9 aa, synthetic construct
GGPGDDTLN

SEQ ID NO: 24712 - protein, 9 aa, synthetic construct
GGPGDDVLF

SEQ ID NO: 24713 - protein, 9 aa, synthetic construct
GGPGDDVIV

SEQ ID NO: 24714 - protein, 9 aa, synthetic construct
GGPGDDVFR

SEQ ID NO: 24715 - protein, 9 aa, synthetic construct
GGAGWDRLH

SEQ ID NO: 24716 - protein, 9 aa, synthetic construct
GGAGWDRMF

SEQ ID NO: 24717 - protein, 9 aa, synthetic construct
GGPGDDTYY

SEQ ID NO: 24718 - protein, 9 aa, synthetic construct
GGPGDDTYL

SEQ ID NO: 24719 - protein, 9 aa, synthetic construct
GGAGWDTFW

SEQ ID NO: 24720 - protein, 9 aa, synthetic construct
GGPGDDTMF

SEQ ID NO: 24721 - protein, 9 aa, synthetic construct
GGAGWDTLE

SEQ ID NO: 24722 - protein, 9 aa, synthetic construct
GGPGDDTLY

SEQ ID NO: 24723 - protein, 9 aa, synthetic construct
GGCGDDVLS

SEQ ID NO: 24724 - protein, 9 aa, synthetic construct
GGPGADRMT

SEQ ID NO: 24725 - protein, 9 aa, synthetic construct
GGPGADRMF

SEQ ID NO: 24726 - protein, 9 aa, synthetic construct
GGPGADRLV

SEQ ID NO: 24727 - protein, 9 aa, synthetic construct
GGNGSDTVI

SEQ ID NO: 24728 - protein, 9 aa, synthetic construct
GGNGSDTMT

SEQ ID NO: 24729 - protein, 9 aa, synthetic construct
GGNGSDTMR

SEQ ID NO: 24730 - protein, 9 aa, synthetic construct
GGGGDDYIM

SEQ ID NO: 24731 - protein, 9 aa, synthetic construct
GGEGDDYIV

SEQ ID NO: 24732 - protein, 9 aa, synthetic construct
GGNGSDTIA

SEQ ID NO: 24733 - protein, 9 aa, synthetic construct
GGNGSDTFA

SEQ ID NO: 24734 - protein, 9 aa, synthetic construct
GGDGADLIL

SEQ ID NO: 24735 - protein, 9 aa, synthetic construct
GGGGDDYIW

SEQ ID NO: 24736 - protein, 9 aa, synthetic construct
GGNGSDSLY

SEQ ID NO: 24737 - protein, 9 aa, synthetic construct
GGDGADLLA

SEQ ID NO: 24738 - protein, 9 aa, synthetic construct
GGNGSDRYV

SEQ ID NO: 24739 - protein, 9 aa, synthetic construct
GGNGSDRYS

SEQ ID NO: 24740 - protein, 9 aa, synthetic construct
GGNGSDRMA

SEQ ID NO: 24741 - protein, 9 aa, synthetic construct
GGNGSDRLR

SEQ ID NO: 24742 - protein, 9 aa, synthetic construct
GGNGSDRLL

SEQ ID NO: 24743 - protein, 9 aa, synthetic construct
GGNGSDQLS

SEQ ID NO: 24744 - protein, 9 aa, synthetic construct
GGNGSDQLF

SEQ ID NO: 24745 - protein, 9 aa, synthetic construct
GGNGSDQIY

SEQ ID NO: 24746 - protein, 9 aa, synthetic construct
GGNGSDQII

SEQ ID NO: 24747 - protein, 9 aa, synthetic construct
GGGGDDYLH

SEQ ID NO: 24748 - protein, 9 aa, synthetic construct
GGDGADLVF

SEQ ID NO: 24749 - protein, 9 aa, synthetic construct
GGDGADLVL

SEQ ID NO: 24750 - protein, 9 aa, synthetic construct
GGDGADLVN

SEQ ID NO: 24751 - protein, 9 aa, synthetic construct
GGDGADLVT

SEQ ID NO: 24752 - protein, 9 aa, synthetic construct
GGDGADLAF

SEQ ID NO: 24753 - protein, 9 aa, synthetic construct
GGNGSDTVS

SEQ ID NO: 24754 - protein, 9 aa, synthetic construct
GGDGADKVF

SEQ ID NO: 24755 - protein, 9 aa, synthetic construct
GGDGADKFD

SEQ ID NO: 24756 - protein, 9 aa, synthetic construct
GGNGTDILF

SEQ ID NO: 24757 - protein, 9 aa, synthetic construct
GGDGADIMG

SEQ ID NO: 24758 - protein, 9 aa, synthetic construct
GGDGADIMV

SEQ ID NO: 24759 - protein, 9 aa, synthetic construct
GGDGADIVD

SEQ ID NO: 24760 - protein, 9 aa, synthetic construct
GGDGADIVE

SEQ ID NO: 24761 - protein, 9 aa, synthetic construct
GGDGADIVI

SEQ ID NO: 24762 - protein, 9 aa, synthetic construct
GGDGADIVS

SEQ ID NO: 24763 - protein, 9 aa, synthetic construct
GGGGDDWLQ

SEQ ID NO: 24764 - protein, 9 aa, synthetic construct
GGGGDDWLS

SEQ ID NO: 24765 - protein, 9 aa, synthetic construct
GGNGSDYLN

SEQ ID NO: 24766 - protein, 9 aa, synthetic construct
GGGGDDWLV

SEQ ID NO: 24767 - protein, 9 aa, synthetic construct
GGNGSDYAE

SEQ ID NO: 24768 - protein, 9 aa, synthetic construct
GGNGSDTYH

SEQ ID NO: 24769 - protein, 9 aa, synthetic construct
GGDGADKFI

SEQ ID NO: 24770 - protein, 9 aa, synthetic construct
GGGGDDWMD

SEQ ID NO: 24771 - protein, 9 aa, synthetic construct
GGDGADKID

SEQ ID NO: 24772 - protein, 9 aa, synthetic construct
GGNGSDVLV

SEQ ID NO: 24773 - protein, 9 aa, synthetic construct
GGNGSDVLE

SEQ ID NO: 24774 - protein, 9 aa, synthetic construct
GGNGSDVLD

SEQ ID NO: 24775 - protein, 9 aa, synthetic construct
GGDGADKLI

SEQ ID NO: 24776 - protein, 9 aa, synthetic construct
GGNGSDVFV

SEQ ID NO: 24777 - protein, 9 aa, synthetic construct
GGDGADKLS

SEQ ID NO: 24778 - protein, 9 aa, synthetic construct
GGNGSDTYS

SEQ ID NO: 24779 - protein, 9 aa, synthetic construct
GGDGADKLW

SEQ ID NO: 24780 - protein, 9 aa, synthetic construct
GGNGSDMII

SEQ ID NO: 24781 - protein, 9 aa, synthetic construct
GGDGADMFR

SEQ ID NO: 24782 - protein, 9 aa, synthetic construct
GGNGSDLIN

SEQ ID NO: 24783 - protein, 9 aa, synthetic construct
GGDGADQIW

SEQ ID NO: 24784 - protein, 9 aa, synthetic construct
GGNGSDALT

SEQ ID NO: 24785 - protein, 9 aa, synthetic construct
GGNGSDALN

SEQ ID NO: 24786 - protein, 9 aa, synthetic construct
GGNGSDAIT

SEQ ID NO: 24787 - protein, 9 aa, synthetic construct
GGGGEDAFV

SEQ ID NO: 24788 - protein, 9 aa, synthetic construct
GGGGEDAIN

SEQ ID NO: 24789 - protein, 9 aa, synthetic construct
GGGGEDALL

SEQ ID NO: 24790 - protein, 9 aa, synthetic construct
GGNGRDVLT

SEQ ID NO: 24791 - protein, 9 aa, synthetic construct
GGNGRDVLR

SEQ ID NO: 24792 - protein, 9 aa, synthetic construct
GGNGRDVLK

SEQ ID NO: 24793 - protein, 9 aa, synthetic construct
GGEGDDWVL

SEQ ID NO: 24794 - protein, 9 aa, synthetic construct
GGNGRDVLF

SEQ ID NO: 24795 - protein, 9 aa, synthetic construct
GGNGRDVFL

SEQ ID NO: 24796 - protein, 9 aa, synthetic construct
GGDGADNLM

SEQ ID NO: 24797 - protein, 9 aa, synthetic construct
GGNGRDTMH

SEQ ID NO: 24798 - protein, 9 aa, synthetic construct
GGNGRDTLR

SEQ ID NO: 24799 - protein, 9 aa, synthetic construct
GGDGADQLI

SEQ ID NO: 24800 - protein, 9 aa, synthetic construct
GGNGRDTLK

SEQ ID NO: 24801 - protein, 9 aa, synthetic construct
GGDGADQLR

SEQ ID NO: 24802 - protein, 9 aa, synthetic construct
GGDGADQLW

SEQ ID NO: 24803 - protein, 9 aa, synthetic construct
GGNGRDTAS

SEQ ID NO: 24804 - protein, 9 aa, synthetic construct
GGNGRDTAD

SEQ ID NO: 24805 - protein, 9 aa, synthetic construct
GGEGDDWMH

SEQ ID NO: 24806 - protein, 9 aa, synthetic construct
GGNGRDSLS

SEQ ID NO: 24807 - protein, 9 aa, synthetic construct
GGEGDDWLY

SEQ ID NO: 24808 - protein, 9 aa, synthetic construct
GGDGADNLT

SEQ ID NO: 24809 - protein, 9 aa, synthetic construct
GGDGADNLI

SEQ ID NO: 24810 - protein, 9 aa, synthetic construct
GGNGSDLIF

SEQ ID NO: 24811 - protein, 9 aa, synthetic construct
GGGGDDYVA

SEQ ID NO: 24812 - protein, 9 aa, synthetic construct
GGNGSDLFV

SEQ ID NO: 24813 - protein, 9 aa, synthetic construct
GGDGADMID

SEQ ID NO: 24814 - protein, 9 aa, synthetic construct
GGDGADMIN

SEQ ID NO: 24815 - protein, 9 aa, synthetic construct
GGGGDDYLQ

SEQ ID NO: 24816 - protein, 9 aa, synthetic construct
GGEGDDYIF

SEQ ID NO: 24817 - protein, 9 aa, synthetic construct
GGNGSDKIY

SEQ ID NO: 24818 - protein, 9 aa, synthetic construct
GGNGSDKIR

SEQ ID NO: 24819 - protein, 9 aa, synthetic construct
GGNGSDILI

SEQ ID NO: 24820 - protein, 9 aa, synthetic construct
GGDGADMLF

SEQ ID NO: 24821 - protein, 9 aa, synthetic construct
GGNGSDIFV

SEQ ID NO: 24822 - protein, 9 aa, synthetic construct
GGNGSDHLY

SEQ ID NO: 24823 - protein, 9 aa, synthetic construct
GGNGSDGLN

SEQ ID NO: 24824 - protein, 9 aa, synthetic construct
GGDGADNLA

SEQ ID NO: 24825 - protein, 9 aa, synthetic construct
GGNGSDFLY

SEQ ID NO: 24826 - protein, 9 aa, synthetic construct
GGDGADMLT

SEQ ID NO: 24827 - protein, 9 aa, synthetic construct
GGDGADMLV

SEQ ID NO: 24828 - protein, 9 aa, synthetic construct
GGDGADNAS

SEQ ID NO: 24829 - protein, 9 aa, synthetic construct
GGNGSDFAD

SEQ ID NO: 24830 - protein, 9 aa, synthetic construct
GGNGSDEMH

SEQ ID NO: 24831 - protein, 9 aa, synthetic construct
GGDGADNIQ

SEQ ID NO: 24832 - protein, 9 aa, synthetic construct
GGNGSDELI

SEQ ID NO: 24833 - protein, 9 aa, synthetic construct
GGNGSDELF

SEQ ID NO: 24834 - protein, 9 aa, synthetic construct
GGDGADNIS

SEQ ID NO: 24835 - protein, 9 aa, synthetic construct
GGNGSDEIE

SEQ ID NO: 24836 - protein, 9 aa, synthetic construct
GGNGTDLLK

SEQ ID NO: 24837 - protein, 9 aa, synthetic construct
GGNGTDLLV

SEQ ID NO: 24838 - protein, 9 aa, synthetic construct
GGDGADILH

SEQ ID NO: 24839 - protein, 9 aa, synthetic construct
GGDGADEFF

SEQ ID NO: 24840 - protein, 9 aa, synthetic construct
GGPGADHLV

SEQ ID NO: 24841 - protein, 9 aa, synthetic construct
GGPGADHLD

SEQ ID NO: 24842 - protein, 9 aa, synthetic construct
GGPGADHIN

SEQ ID NO: 24843 - protein, 9 aa, synthetic construct
GGDGADDLG

SEQ ID NO: 24844 - protein, 9 aa, synthetic construct
GGDGADDLH

SEQ ID NO: 24845 - protein, 9 aa, synthetic construct
GGDGADDLL

SEQ ID NO: 24846 - protein, 9 aa, synthetic construct
GGPGADAMI

SEQ ID NO: 24847 - protein, 9 aa, synthetic construct
GGDGADDLY

SEQ ID NO: 24848 - protein, 9 aa, synthetic construct
GGPGADAFD

SEQ ID NO: 24849 - protein, 9 aa, synthetic construct
GGEGEDALI

SEQ ID NO: 24850 - protein, 9 aa, synthetic construct
GGNGYDVIF

SEQ ID NO: 24851 - protein, 9 aa, synthetic construct
GGNGYDTLS

SEQ ID NO: 24852 - protein, 9 aa, synthetic construct
GGPGADIFV

SEQ ID NO: 24853 - protein, 9 aa, synthetic construct
GGNGYDSLS

SEQ ID NO: 24854 - protein, 9 aa, synthetic construct
GGNGYDRVN

SEQ ID NO: 24855 - protein, 9 aa, synthetic construct
GGDGADEIR

SEQ ID NO: 24856 - protein, 9 aa, synthetic construct
GGNGYDQIQ

SEQ ID NO: 24857 - protein, 9 aa, synthetic construct
GGDGADELD

SEQ ID NO: 24858 - protein, 9 aa, synthetic construct
GGNGYDILN

SEQ ID NO: 24859 - protein, 9 aa, synthetic construct
GGNGYDGLK

SEQ ID NO: 24860 - protein, 9 aa, synthetic construct
GGDGADELL

SEQ ID NO: 24861 - protein, 9 aa, synthetic construct
GGNGWDYLI

SEQ ID NO: 24862 - protein, 9 aa, synthetic construct
GGNGWDYAL

SEQ ID NO: 24863 - protein, 9 aa, synthetic construct
GGNGWDVAS

SEQ ID NO: 24864 - protein, 9 aa, synthetic construct
GGDGADDIS

SEQ ID NO: 24865 - protein, 9 aa, synthetic construct
GGDGADDID

SEQ ID NO: 24866 - protein, 9 aa, synthetic construct
GGDGADELW

SEQ ID NO: 24867 - protein, 9 aa, synthetic construct
GGGGDDTYT

SEQ ID NO: 24868 - protein, 9 aa, synthetic construct
GGPGADRLT

SEQ ID NO: 24869 - protein, 9 aa, synthetic construct
GGPGADRLS

SEQ ID NO: 24870 - protein, 9 aa, synthetic construct
GGPGADRLN

SEQ ID NO: 24871 - protein, 9 aa, synthetic construct
GGGGDDTVS

SEQ ID NO: 24872 - protein, 9 aa, synthetic construct
GGGGDDTVW

SEQ ID NO: 24873 - protein, 9 aa, synthetic construct
GGPGADRFI

SEQ ID NO: 24874 - protein, 9 aa, synthetic construct
GGPGADQLY

SEQ ID NO: 24875 - protein, 9 aa, synthetic construct
GGDGADAIA

SEQ ID NO: 24876 - protein, 9 aa, synthetic construct
GGPGADNMT

SEQ ID NO: 24877 - protein, 9 aa, synthetic construct
GGGGDDTYK

SEQ ID NO: 24878 - protein, 9 aa, synthetic construct
GGPGADNFV

SEQ ID NO: 24879 - protein, 9 aa, synthetic construct
GGPGADMLD

SEQ ID NO: 24880 - protein, 9 aa, synthetic construct
GGPGADILD

SEQ ID NO: 24881 - protein, 9 aa, synthetic construct
GGPGADLLW

SEQ ID NO: 24882 - protein, 9 aa, synthetic construct
GGDGADALI

SEQ ID NO: 24883 - protein, 9 aa, synthetic construct
GGGGDDVFD

SEQ ID NO: 24884 - protein, 9 aa, synthetic construct
GGPGADLLK

SEQ ID NO: 24885 - protein, 9 aa, synthetic construct
GGDGADAVS

SEQ ID NO: 24886 - protein, 9 aa, synthetic construct
GGDGADAYV

SEQ ID NO: 24887 - protein, 9 aa, synthetic construct
GGPGADIVN

SEQ ID NO: 24888 - protein, 9 aa, synthetic construct
GGDGADCLI

SEQ ID NO: 24889 - protein, 9 aa, synthetic construct
GGDGADCLN

SEQ ID NO: 24890 - protein, 9 aa, synthetic construct
GGPGADILN

SEQ ID NO: 24891 - protein, 9 aa, synthetic construct
GGPGADILG

SEQ ID NO: 24892 - protein, 9 aa, synthetic construct
GGDGADELT

SEQ ID NO: 24893 - protein, 9 aa, synthetic construct
GGNGWDRLS

SEQ ID NO: 24894 - protein, 9 aa, synthetic construct
GGNGTDQLN

SEQ ID NO: 24895 - protein, 9 aa, synthetic construct
GGGGDDWIL

SEQ ID NO: 24896 - protein, 9 aa, synthetic construct
GGNGVDAIQ

SEQ ID NO: 24897 - protein, 9 aa, synthetic construct
GGEGDDYLW

SEQ ID NO: 24898 - protein, 9 aa, synthetic construct
GGDGADHLY

SEQ ID NO: 24899 - protein, 9 aa, synthetic construct
GGEGDDYLV

SEQ ID NO: 24900 - protein, 9 aa, synthetic construct
GGNGTDYIE

SEQ ID NO: 24901 - protein, 9 aa, synthetic construct
GGNGTDVVS

SEQ ID NO: 24902 - protein, 9 aa, synthetic construct
GGNGTDVLD

SEQ ID NO: 24903 - protein, 9 aa, synthetic construct
GGNGTDVIY

SEQ ID NO: 24904 - protein, 9 aa, synthetic construct
GGDGADIFI

SEQ ID NO: 24905 - protein, 9 aa, synthetic construct
GGDGADIFL

SEQ ID NO: 24906 - protein, 9 aa, synthetic construct
GGNGTDTLV

SEQ ID NO: 24907 - protein, 9 aa, synthetic construct
GGDGADIID

SEQ ID NO: 24908 - protein, 9 aa, synthetic construct
GGDGADHLF

SEQ ID NO: 24909 - protein, 9 aa, synthetic construct
GGDGADIIF

SEQ ID NO: 24910 - protein, 9 aa, synthetic construct
GGNGTDTAT

SEQ ID NO: 24911 - protein, 9 aa, synthetic construct
GGDGADIIN

SEQ ID NO: 24912 - protein, 9 aa, synthetic construct
GGNGTDTAI

SEQ ID NO: 24913 - protein, 9 aa, synthetic construct
GGDGADIIQ

SEQ ID NO: 24914 - protein, 9 aa, synthetic construct
GGGGDDWIR

SEQ ID NO: 24915 - protein, 9 aa, synthetic construct
GGDGADIIS

SEQ ID NO: 24916 - protein, 9 aa, synthetic construct
GGNGTDSID

SEQ ID NO: 24917 - protein, 9 aa, synthetic construct
GGGGDDWIY

SEQ ID NO: 24918 - protein, 9 aa, synthetic construct
GGNGTDRLI

SEQ ID NO: 24919 - protein, 9 aa, synthetic construct
GGNGTDRLF

SEQ ID NO: 24920 - protein, 9 aa, synthetic construct
GGEGDDYME

SEQ ID NO: 24921 - protein, 9 aa, synthetic construct
GGGGDDVYL

SEQ ID NO: 24922 - protein, 9 aa, synthetic construct
GGGGDDVLH

SEQ ID NO: 24923 - protein, 9 aa, synthetic construct
GGNGVDTVL

SEQ ID NO: 24924 - protein, 9 aa, synthetic construct
GGDGADFAS

SEQ ID NO: 24925 - protein, 9 aa, synthetic construct
GGNGWDKLF

SEQ ID NO: 24926 - protein, 9 aa, synthetic construct
GGNGWDILK

SEQ ID NO: 24927 - protein, 9 aa, synthetic construct
GGDGADFIL

SEQ ID NO: 24928 - protein, 9 aa, synthetic construct
GGNGWDELW

SEQ ID NO: 24929 - protein, 9 aa, synthetic construct
GGDGADFIS

SEQ ID NO: 24930 - protein, 9 aa, synthetic construct
GGDGADFLA

SEQ ID NO: 24931 - protein, 9 aa, synthetic construct
GGNGVDYAT

SEQ ID NO: 24932 - protein, 9 aa, synthetic construct
GGNGVDVLN

SEQ ID NO: 24933 - protein, 9 aa, synthetic construct
GGNGVDTYE

SEQ ID NO: 24934 - protein, 9 aa, synthetic construct
GGNGVDTVM

SEQ ID NO: 24935 - protein, 9 aa, synthetic construct
GGGGDDVMD

SEQ ID NO: 24936 - protein, 9 aa, synthetic construct
GGNGVDLLQ

SEQ ID NO: 24937 - protein, 9 aa, synthetic construct
GGNGVDTLD

SEQ ID NO: 24938 - protein, 9 aa, synthetic construct
GGEGEDALF

SEQ ID NO: 24939 - protein, 9 aa, synthetic construct
GGNGVDTIY

SEQ ID NO: 24940 - protein, 9 aa, synthetic construct
GGNGVDTIS

SEQ ID NO: 24941 - protein, 9 aa, synthetic construct
GGNGVDTFV

SEQ ID NO: 24942 - protein, 9 aa, synthetic construct
GGNGVDTFI

SEQ ID NO: 24943 - protein, 9 aa, synthetic construct
GGDGADFVR

SEQ ID NO: 24944 - protein, 9 aa, synthetic construct
GGNGVDSLN

SEQ ID NO: 24945 - protein, 9 aa, synthetic construct
GGDGADGIF

SEQ ID NO: 24946 - protein, 9 aa, synthetic construct
GGGGDDVVA

SEQ ID NO: 24947 - protein, 9 aa, synthetic construct
GGGGDDVVS

SEQ ID NO: 24948 - protein, 9 aa, synthetic construct
GGPGHDQLL

SEQ ID NO: 24949 - protein, 9 aa, synthetic construct
GGPGHDRLD

SEQ ID NO: 24950 - protein, 9 aa, synthetic construct
GGQGDDAIT

SEQ ID NO: 24951 - protein, 9 aa, synthetic construct
GGPGYDRLE

SEQ ID NO: 24952 - protein, 9 aa, synthetic construct
GGEGFDILR

SEQ ID NO: 24953 - protein, 9 aa, synthetic construct
GGAGTDSIE

SEQ ID NO: 24954 - protein, 9 aa, synthetic construct
GGPGTDLLD

SEQ ID NO: 24955 - protein, 9 aa, synthetic construct
GGPGTDIII

SEQ ID NO: 24956 - protein, 9 aa, synthetic construct
GGAGTDSLE

SEQ ID NO: 24957 - protein, 9 aa, synthetic construct
GGAGTDSLF

SEQ ID NO: 24958 - protein, 9 aa, synthetic construct
GGAGTDSLR

SEQ ID NO: 24959 - protein, 9 aa, synthetic construct
GGPGTDELT

SEQ ID NO: 24960 - protein, 9 aa, synthetic construct
GGPGTDAMD

SEQ ID NO: 24961 - protein, 9 aa, synthetic construct
GGAGTDSMN

SEQ ID NO: 24962 - protein, 9 aa, synthetic construct
GGAGTDSMV

SEQ ID NO: 24963 - protein, 9 aa, synthetic construct
GGGGDDIAT

SEQ ID NO: 24964 - protein, 9 aa, synthetic construct
GGPGSDVVD

SEQ ID NO: 24965 - protein, 9 aa, synthetic construct
GGAGTDSVF

SEQ ID NO: 24966 - protein, 9 aa, synthetic construct
GGAGTDSVT

SEQ ID NO: 24967 - protein, 9 aa, synthetic construct
GGPGSDVLI

SEQ ID NO: 24968 - protein, 9 aa, synthetic construct
GGPGSDVID

SEQ ID NO: 24969 - protein, 9 aa, synthetic construct
GGPGSDTYI

SEQ ID NO: 24970 - protein, 9 aa, synthetic construct
GGAGTDTAG

SEQ ID NO: 24971 - protein, 9 aa, synthetic construct
GGGGDDIFC

SEQ ID NO: 24972 - protein, 9 aa, synthetic construct
GGAGTDTAK

SEQ ID NO: 24973 - protein, 9 aa, synthetic construct
GGAGTDTAN

SEQ ID NO: 24974 - protein, 9 aa, synthetic construct
GGPGSDTLF

SEQ ID NO: 24975 - protein, 9 aa, synthetic construct
GGGGDDIFL

SEQ ID NO: 24976 - protein, 9 aa, synthetic construct
GGPGSDTIY

SEQ ID NO: 24977 - protein, 9 aa, synthetic construct
GGPGTDNIY

SEQ ID NO: 24978 - protein, 9 aa, synthetic construct
GGGGDDHLH

SEQ ID NO: 24979 - protein, 9 aa, synthetic construct
GGGGDDHLF

SEQ ID NO: 24980 - protein, 9 aa, synthetic construct
GGPGVDRLF

SEQ ID NO: 24981 - protein, 9 aa, synthetic construct
GGPGYDLMY

SEQ ID NO: 24982 - protein, 9 aa, synthetic construct
GGAGTDQMQ

SEQ ID NO: 24983 - protein, 9 aa, synthetic construct
GGPGYDFLE

SEQ ID NO: 24984 - protein, 9 aa, synthetic construct
GGPGWDYLV

SEQ ID NO: 24985 - protein, 9 aa, synthetic construct
GGPGWDTAI

SEQ ID NO: 24986 - protein, 9 aa, synthetic construct
GGGGDDGYI

SEQ ID NO: 24987 - protein, 9 aa, synthetic construct
GGAGTDRFD

SEQ ID NO: 24988 - protein, 9 aa, synthetic construct
GGAGTDRFY

SEQ ID NO: 24989 - protein, 9 aa, synthetic construct
GGAGTDRID

SEQ ID NO: 24990 - protein, 9 aa, synthetic construct
GGAGTDRIE

SEQ ID NO: 24991 - protein, 9 aa, synthetic construct
GGAGTDRIW

SEQ ID NO: 24992 - protein, 9 aa, synthetic construct
GGPGVDRAF

SEQ ID NO: 24993 - protein, 9 aa, synthetic construct
GGAGTDRVT

SEQ ID NO: 24994 - protein, 9 aa, synthetic construct
GGPGVDLMA

SEQ ID NO: 24995 - protein, 9 aa, synthetic construct
GGPGVDIMT

SEQ ID NO: 24996 - protein, 9 aa, synthetic construct
GGGGDDHII

SEQ ID NO: 24997 - protein, 9 aa, synthetic construct
GGPGTDVLD

SEQ ID NO: 24998 - protein, 9 aa, synthetic construct
GGPGTDVFL

SEQ ID NO: 24999 - protein, 9 aa, synthetic construct
GGGGDDHIL

SEQ ID NO: 25000 - protein, 9 aa, synthetic construct
GGGGDDHIN

SEQ ID NO: 25001 - protein, 9 aa, synthetic construct
GGGGDDHIT

SEQ ID NO: 25002 - protein, 9 aa, synthetic construct
GGGGDDHLA

SEQ ID NO: 25003 - protein, 9 aa, synthetic construct
GGGGDDHLD

SEQ ID NO: 25004 - protein, 9 aa, synthetic construct
GGPGTDTIY

SEQ ID NO: 25005 - protein, 9 aa, synthetic construct
GGPGSDTIR

SEQ ID NO: 25006 - protein, 9 aa, synthetic construct
GGPGSDTIN

SEQ ID NO: 25007 - protein, 9 aa, synthetic construct
GGPGSDTID

SEQ ID NO: 25008 - protein, 9 aa, synthetic construct
GGPGRDRMY

SEQ ID NO: 25009 - protein, 9 aa, synthetic construct
GGAGTDTVY

SEQ ID NO: 25010 - protein, 9 aa, synthetic construct
GGPGRDTLW

SEQ ID NO: 25011 - protein, 9 aa, synthetic construct
GGAGTDTYV

SEQ ID NO: 25012 - protein, 9 aa, synthetic construct
GGPGRDTLQ

SEQ ID NO: 25013 - protein, 9 aa, synthetic construct
GGAGTDTYY

SEQ ID NO: 25014 - protein, 9 aa, synthetic construct
GGPGRDTLK

SEQ ID NO: 25015 - protein, 9 aa, synthetic construct
GGPGRDTLH

SEQ ID NO: 25016 - protein, 9 aa, synthetic construct
GGAGTDVAD

SEQ ID NO: 25017 - protein, 9 aa, synthetic construct
GGPGRDTII

SEQ ID NO: 25018 - protein, 9 aa, synthetic construct
GGAGTDVAI

SEQ ID NO: 25019 - protein, 9 aa, synthetic construct
GGEGFDFIA

SEQ ID NO: 25020 - protein, 9 aa, synthetic construct
GGPGRDRIH

SEQ ID NO: 25021 - protein, 9 aa, synthetic construct
GGPGRDVIK

SEQ ID NO: 25022 - protein, 9 aa, synthetic construct
GGAGTDVIL

SEQ ID NO: 25023 - protein, 9 aa, synthetic construct
GGAGTDVIY

SEQ ID NO: 25024 - protein, 9 aa, synthetic construct
GGAGTDVLF

SEQ ID NO: 25025 - protein, 9 aa, synthetic construct
GGGGDDILC

SEQ ID NO: 25026 - protein, 9 aa, synthetic construct
GGPGRDLLI

SEQ ID NO: 25027 - protein, 9 aa, synthetic construct
GGAGTDVMA

SEQ ID NO: 25028 - protein, 9 aa, synthetic construct
GGAGTDWAN

SEQ ID NO: 25029 - protein, 9 aa, synthetic construct
GGPGRDILR

SEQ ID NO: 25030 - protein, 9 aa, synthetic construct
GGAGNDVFM

SEQ ID NO: 25031 - protein, 9 aa, synthetic construct
GGPGRDILD

SEQ ID NO: 25032 - protein, 9 aa, synthetic construct
GGAGTDWID

SEQ ID NO: 25033 - protein, 9 aa, synthetic construct
GGPGRDVID

SEQ ID NO: 25034 - protein, 9 aa, synthetic construct
GGPGRDVIY

SEQ ID NO: 25035 - protein, 9 aa, synthetic construct
GGPGSDTFL

SEQ ID NO: 25036 - protein, 9 aa, synthetic construct
GGPGSDNLQ

SEQ ID NO: 25037 - protein, 9 aa, synthetic construct
GGAGTDTAY

SEQ ID NO: 25038 - protein, 9 aa, synthetic construct
GGAGTDTFA

SEQ ID NO: 25039 - protein, 9 aa, synthetic construct
GGAGTDTFI

SEQ ID NO: 25040 - protein, 9 aa, synthetic construct
GGPGSDSIF

SEQ ID NO: 25041 - protein, 9 aa, synthetic construct
GGAGTDTFL

SEQ ID NO: 25042 - protein, 9 aa, synthetic construct
GGAGTDTFS

SEQ ID NO: 25043 - protein, 9 aa, synthetic construct
GGPGSDRLE

SEQ ID NO: 25044 - protein, 9 aa, synthetic construct
GGAGTDTFT

SEQ ID NO: 25045 - protein, 9 aa, synthetic construct
GGAGTDTIF

SEQ ID NO: 25046 - protein, 9 aa, synthetic construct
GGAGTDTIH

SEQ ID NO: 25047 - protein, 9 aa, synthetic construct
GGPGSDNVE

SEQ ID NO: 25048 - protein, 9 aa, synthetic construct
GGPGSDIFY

SEQ ID NO: 25049 - protein, 9 aa, synthetic construct
GGPGRDVLK

SEQ ID NO: 25050 - protein, 9 aa, synthetic construct
GGPGSDHYR

SEQ ID NO: 25051 - protein, 9 aa, synthetic construct
GGPGSDHLY

SEQ ID NO: 25052 - protein, 9 aa, synthetic construct
GGPGSDFID

SEQ ID NO: 25053 - protein, 9 aa, synthetic construct
GGPGSDALT

SEQ ID NO: 25054 - protein, 9 aa, synthetic construct
GGPGSDAII

SEQ ID NO: 25055 - protein, 9 aa, synthetic construct
GGAGTDTMA

SEQ ID NO: 25056 - protein, 9 aa, synthetic construct
GGAGTDTMN

SEQ ID NO: 25057 - protein, 9 aa, synthetic construct
GGPGRDWLV

SEQ ID NO: 25058 - protein, 9 aa, synthetic construct
GGGGDDIFY

SEQ ID NO: 25059 - protein, 9 aa, synthetic construct
GGPGRDVMV

SEQ ID NO: 25060 - protein, 9 aa, synthetic construct
GGAGTDTMS

SEQ ID NO: 25061 - protein, 9 aa, synthetic construct
GGAGTDQMF

SEQ ID NO: 25062 - protein, 9 aa, synthetic construct
GGAGTDQLY

SEQ ID NO: 25063 - protein, 9 aa, synthetic construct
GGPGHDRLS

SEQ ID NO: 25064 - protein, 9 aa, synthetic construct
GGEGFDLID

SEQ ID NO: 25065 - protein, 9 aa, synthetic construct
GGAGTDIFK

SEQ ID NO: 25066 - protein, 9 aa, synthetic construct
GGGGDDELY

SEQ ID NO: 25067 - protein, 9 aa, synthetic construct
GGQGADTMH

SEQ ID NO: 25068 - protein, 9 aa, synthetic construct
GGEGFDTAV

SEQ ID NO: 25069 - protein, 9 aa, synthetic construct
GGQGADTLW

SEQ ID NO: 25070 - protein, 9 aa, synthetic construct
GGQGADTLQ

SEQ ID NO: 25071 - protein, 9 aa, synthetic construct
GGQGADTLN

SEQ ID NO: 25072 - protein, 9 aa, synthetic construct
GGQGADTLM

SEQ ID NO: 25073 - protein, 9 aa, synthetic construct
GGQGADTLK

SEQ ID NO: 25074 - protein, 9 aa, synthetic construct
GGQGADTLH

SEQ ID NO: 25075 - protein, 9 aa, synthetic construct
GGQGADTLA

SEQ ID NO: 25076 - protein, 9 aa, synthetic construct
GGAGTDILK

SEQ ID NO: 25077 - protein, 9 aa, synthetic construct
GGAGTDILL

SEQ ID NO: 25078 - protein, 9 aa, synthetic construct
GGAGTDILQ

SEQ ID NO: 25079 - protein, 9 aa, synthetic construct
GGQGADTAF

SEQ ID NO: 25080 - protein, 9 aa, synthetic construct
GGGGDDEVA

SEQ ID NO: 25081 - protein, 9 aa, synthetic construct
GGQGADSMW

SEQ ID NO: 25082 - protein, 9 aa, synthetic construct
GGAGTDIMS

SEQ ID NO: 25083 - protein, 9 aa, synthetic construct
GGGGDDFFW

SEQ ID NO: 25084 - protein, 9 aa, synthetic construct
GGAGTDIVS

SEQ ID NO: 25085 - protein, 9 aa, synthetic construct
GGQGADSLE

SEQ ID NO: 25086 - protein, 9 aa, synthetic construct
GGQGADSIY

SEQ ID NO: 25087 - protein, 9 aa, synthetic construct
GGEGFDSLL

SEQ ID NO: 25088 - protein, 9 aa, synthetic construct
GGAGTDKLY

SEQ ID NO: 25089 - protein, 9 aa, synthetic construct
GGAGTDKVS

SEQ ID NO: 25090 - protein, 9 aa, synthetic construct
GGQGADTVS

SEQ ID NO: 25091 - protein, 9 aa, synthetic construct
GGQGADTVV

SEQ ID NO: 25092 - protein, 9 aa, synthetic construct
GGQGADTYH

SEQ ID NO: 25093 - protein, 9 aa, synthetic construct
GGQGADVLV

SEQ ID NO: 25094 - protein, 9 aa, synthetic construct
GGEGFDTLD

SEQ ID NO: 25095 - protein, 9 aa, synthetic construct
GGGGDDEIK

SEQ ID NO: 25096 - protein, 9 aa, synthetic construct
GGGGDDEIN

SEQ ID NO: 25097 - protein, 9 aa, synthetic construct
GGQGADYLR

SEQ ID NO: 25098 - protein, 9 aa, synthetic construct
GGQGADYLK

SEQ ID NO: 25099 - protein, 9 aa, synthetic construct
GGQGADWMV

SEQ ID NO: 25100 - protein, 9 aa, synthetic construct
GGGGDDELA

SEQ ID NO: 25101 - protein, 9 aa, synthetic construct
GGQGADVVR

SEQ ID NO: 25102 - protein, 9 aa, synthetic construct
GGQGADVVQ

SEQ ID NO: 25103 - protein, 9 aa, synthetic construct
GGQGADVVL

SEQ ID NO: 25104 - protein, 9 aa, synthetic construct
GGAGTDHLL

SEQ ID NO: 25105 - protein, 9 aa, synthetic construct
GGQGADVLS

SEQ ID NO: 25106 - protein, 9 aa, synthetic construct
GGQGADTYV

SEQ ID NO: 25107 - protein, 9 aa, synthetic construct
GGQGADVLN

SEQ ID NO: 25108 - protein, 9 aa, synthetic construct
GGQGADVLI

SEQ ID NO: 25109 - protein, 9 aa, synthetic construct
GGQGADVLH

SEQ ID NO: 25110 - protein, 9 aa, synthetic construct
GGAGTDHME

SEQ ID NO: 25111 - protein, 9 aa, synthetic construct
GGQGADVLD

SEQ ID NO: 25112 - protein, 9 aa, synthetic construct
GGQGADVLA

SEQ ID NO: 25113 - protein, 9 aa, synthetic construct
GGQGADVIS

SEQ ID NO: 25114 - protein, 9 aa, synthetic construct
GGGGDDELI

SEQ ID NO: 25115 - protein, 9 aa, synthetic construct
GGQGADVIL

SEQ ID NO: 25116 - protein, 9 aa, synthetic construct
GGEGFDTFV

SEQ ID NO: 25117 - protein, 9 aa, synthetic construct
GGQGADVFI

SEQ ID NO: 25118 - protein, 9 aa, synthetic construct
GGGGDDFIV

SEQ ID NO: 25119 - protein, 9 aa, synthetic construct
GGQGADRLS

SEQ ID NO: 25120 - protein, 9 aa, synthetic construct
GGGGDDFIY

SEQ ID NO: 25121 - protein, 9 aa, synthetic construct
GGAGTDQLF

SEQ ID NO: 25122 - protein, 9 aa, synthetic construct
GGAGTDMLY

SEQ ID NO: 25123 - protein, 9 aa, synthetic construct
GGEGFDQIN

SEQ ID NO: 25124 - protein, 9 aa, synthetic construct
GGAGTDNLR

SEQ ID NO: 25125 - protein, 9 aa, synthetic construct
GGQGADFIA

SEQ ID NO: 25126 - protein, 9 aa, synthetic construct
GGAGTDNVD

SEQ ID NO: 25127 - protein, 9 aa, synthetic construct
GGQGADELT

SEQ ID NO: 25128 - protein, 9 aa, synthetic construct
GGQGADELR

SEQ ID NO: 25129 - protein, 9 aa, synthetic construct
GGEGFDLLY

SEQ ID NO: 25130 - protein, 9 aa, synthetic construct
GGAGTDQLD

SEQ ID NO: 25131 - protein, 9 aa, synthetic construct
GGAGTDQLE

SEQ ID NO: 25132 - protein, 9 aa, synthetic construct
GGQGADDLS

SEQ ID NO: 25133 - protein, 9 aa, synthetic construct
GGGGDDGLF

SEQ ID NO: 25134 - protein, 9 aa, synthetic construct
GGQGADHMV

SEQ ID NO: 25135 - protein, 9 aa, synthetic construct
GGQGADDIW

SEQ ID NO: 25136 - protein, 9 aa, synthetic construct
GGQGADAMS

SEQ ID NO: 25137 - protein, 9 aa, synthetic construct
GGAGTDQLI

SEQ ID NO: 25138 - protein, 9 aa, synthetic construct
GGQGADAMF

SEQ ID NO: 25139 - protein, 9 aa, synthetic construct
GGAGTDQLL

SEQ ID NO: 25140 - protein, 9 aa, synthetic construct
GGQGADALS

SEQ ID NO: 25141 - protein, 9 aa, synthetic construct
GGGGDDGLH

SEQ ID NO: 25142 - protein, 9 aa, synthetic construct
GGQGADALD

SEQ ID NO: 25143 - protein, 9 aa, synthetic construct
GGAGTDQLS

SEQ ID NO: 25144 - protein, 9 aa, synthetic construct
GGPGYDTLW

SEQ ID NO: 25145 - protein, 9 aa, synthetic construct
GGAGTDQLT

SEQ ID NO: 25146 - protein, 9 aa, synthetic construct
GGAGTDMLA

SEQ ID NO: 25147 - protein, 9 aa, synthetic construct
GGQGADILD

SEQ ID NO: 25148 - protein, 9 aa, synthetic construct
GGQGADQVL

SEQ ID NO: 25149 - protein, 9 aa, synthetic construct
GGAGTDLMV

SEQ ID NO: 25150 - protein, 9 aa, synthetic construct
GGQGADQMT

SEQ ID NO: 25151 - protein, 9 aa, synthetic construct
GGQGADQLI

SEQ ID NO: 25152 - protein, 9 aa, synthetic construct
GGAGTDLIN

SEQ ID NO: 25153 - protein, 9 aa, synthetic construct
GGAGTDLLA

SEQ ID NO: 25154 - protein, 9 aa, synthetic construct
GGQGADNLV

SEQ ID NO: 25155 - protein, 9 aa, synthetic construct
GGAGTDLLS

SEQ ID NO: 25156 - protein, 9 aa, synthetic construct
GGAGTDLLT

SEQ ID NO: 25157 - protein, 9 aa, synthetic construct
GGQGADMLD

SEQ ID NO: 25158 - protein, 9 aa, synthetic construct
GGGGDDFLR

SEQ ID NO: 25159 - protein, 9 aa, synthetic construct
GGQGADLMM

SEQ ID NO: 25160 - protein, 9 aa, synthetic construct
GGGGDDFLV

SEQ ID NO: 25161 - protein, 9 aa, synthetic construct
GGQGADLLS

SEQ ID NO: 25162 - protein, 9 aa, synthetic construct
GGQGADILG

SEQ ID NO: 25163 - protein, 9 aa, synthetic construct
GGQGADLIY

SEQ ID NO: 25164 - protein, 9 aa, synthetic construct
GGQGADLIV

SEQ ID NO: 25165 - protein, 9 aa, synthetic construct
GGQGADLFR

SEQ ID NO: 25166 - protein, 9 aa, synthetic construct
GGQGADLFL

SEQ ID NO: 25167 - protein, 9 aa, synthetic construct
GGQGADKLY

SEQ ID NO: 25168 - protein, 9 aa, synthetic construct
GGQGADKLT

SEQ ID NO: 25169 - protein, 9 aa, synthetic construct
GGQGADKLS

SEQ ID NO: 25170 - protein, 9 aa, synthetic construct
GGEGFDRLE

SEQ ID NO: 25171 - protein, 9 aa, synthetic construct
GGQGADKFQ

SEQ ID NO: 25172 - protein, 9 aa, synthetic construct
GGQGADIVN

SEQ ID NO: 25173 - protein, 9 aa, synthetic construct
GGQGADILR

SEQ ID NO: 25174 - protein, 9 aa, synthetic construct
GGAGTDYAS

SEQ ID NO: 25175 - protein, 9 aa, synthetic construct
GGGGDDIVD

SEQ ID NO: 25176 - protein, 9 aa, synthetic construct
GGAGTDYIE

SEQ ID NO: 25177 - protein, 9 aa, synthetic construct
GGAGTDYIY

SEQ ID NO: 25178 - protein, 9 aa, synthetic construct
GGAGVDNLF

SEQ ID NO: 25179 - protein, 9 aa, synthetic construct
GGEGEDTLR

SEQ ID NO: 25180 - protein, 9 aa, synthetic construct
GGPGNDHIT

SEQ ID NO: 25181 - protein, 9 aa, synthetic construct
GGAGVDNLT

SEQ ID NO: 25182 - protein, 9 aa, synthetic construct
GGPGNDHFT

SEQ ID NO: 25183 - protein, 9 aa, synthetic construct
GGPGNDGLY

SEQ ID NO: 25184 - protein, 9 aa, synthetic construct
GGGGDDMIK

SEQ ID NO: 25185 - protein, 9 aa, synthetic construct
GGAGVDQID

SEQ ID NO: 25186 - protein, 9 aa, synthetic construct
GGPGNDFLD

SEQ ID NO: 25187 - protein, 9 aa, synthetic construct
GGPGNDFLA

SEQ ID NO: 25188 - protein, 9 aa, synthetic construct
GGGGDDMIT

SEQ ID NO: 25189 - protein, 9 aa, synthetic construct
GGPGNDFIQ

SEQ ID NO: 25190 - protein, 9 aa, synthetic construct
GGPGNDFID

SEQ ID NO: 25191 - protein, 9 aa, synthetic construct
GGPGNDELS

SEQ ID NO: 25192 - protein, 9 aa, synthetic construct
GGPGNDELK

SEQ ID NO: 25193 - protein, 9 aa, synthetic construct
GGPGNDELI

SEQ ID NO: 25194 - protein, 9 aa, synthetic construct
GGPGNDEIW

SEQ ID NO: 25195 - protein, 9 aa, synthetic construct
GGPGNDEIH

SEQ ID NO: 25196 - protein, 9 aa, synthetic construct
GGPGNDDLY

SEQ ID NO: 25197 - protein, 9 aa, synthetic construct
GGPGNDDLW

SEQ ID NO: 25198 - protein, 9 aa, synthetic construct
GGAGVDQVR

SEQ ID NO: 25199 - protein, 9 aa, synthetic construct
GGAGVDQVS

SEQ ID NO: 25200 - protein, 9 aa, synthetic construct
GGAGVDRAD

SEQ ID NO: 25201 - protein, 9 aa, synthetic construct
GGGGDDMLV

SEQ ID NO: 25202 - protein, 9 aa, synthetic construct
GGAGVDRAS

SEQ ID NO: 25203 - protein, 9 aa, synthetic construct
GGAGVDNLD

SEQ ID NO: 25204 - protein, 9 aa, synthetic construct
GGAGVDNIV

SEQ ID NO: 25205 - protein, 9 aa, synthetic construct
GGAGVDNIT

SEQ ID NO: 25206 - protein, 9 aa, synthetic construct
GGPGNDLIE

SEQ ID NO: 25207 - protein, 9 aa, synthetic construct
GGPGNDMIY

SEQ ID NO: 25208 - protein, 9 aa, synthetic construct
GGAGVDLLR

SEQ ID NO: 25209 - protein, 9 aa, synthetic construct
GGGGDDLMY

SEQ ID NO: 25210 - protein, 9 aa, synthetic construct
GGPGNDLVS

SEQ ID NO: 25211 - protein, 9 aa, synthetic construct
GGPGNDLMV

SEQ ID NO: 25212 - protein, 9 aa, synthetic construct
GGGGDDLVD

SEQ ID NO: 25213 - protein, 9 aa, synthetic construct
GGGGDDLVF

SEQ ID NO: 25214 - protein, 9 aa, synthetic construct
GGGGDDLVR

SEQ ID NO: 25215 - protein, 9 aa, synthetic construct
GGAGVDMAV

SEQ ID NO: 25216 - protein, 9 aa, synthetic construct
GGPGNDLIR

SEQ ID NO: 25217 - protein, 9 aa, synthetic construct
GGAGVDMLD

SEQ ID NO: 25218 - protein, 9 aa, synthetic construct
GGPGNDLID

SEQ ID NO: 25219 - protein, 9 aa, synthetic construct
GGPGNDIMI

SEQ ID NO: 25220 - protein, 9 aa, synthetic construct
GGPGNDLFY

SEQ ID NO: 25221 - protein, 9 aa, synthetic construct
GGPGNDKLT

SEQ ID NO: 25222 - protein, 9 aa, synthetic construct
GGPGNDKLR

SEQ ID NO: 25223 - protein, 9 aa, synthetic construct
GGPGNDKLQ

SEQ ID NO: 25224 - protein, 9 aa, synthetic construct
GGAGVDMLS

SEQ ID NO: 25225 - protein, 9 aa, synthetic construct
GGPGNDKLD

SEQ ID NO: 25226 - protein, 9 aa, synthetic construct
GGGGDDLYI

SEQ ID NO: 25227 - protein, 9 aa, synthetic construct
GGPGNDKID

SEQ ID NO: 25228 - protein, 9 aa, synthetic construct
GGPGNDIYW

SEQ ID NO: 25229 - protein, 9 aa, synthetic construct
GGPGNDIYV

SEQ ID NO: 25230 - protein, 9 aa, synthetic construct
GGPGNDIMY

SEQ ID NO: 25231 - protein, 9 aa, synthetic construct
GGGGDDMLY

SEQ ID NO: 25232 - protein, 9 aa, synthetic construct
GGPGNDALF

SEQ ID NO: 25233 - protein, 9 aa, synthetic construct
GGEGEDTLI

SEQ ID NO: 25234 - protein, 9 aa, synthetic construct
GGAGVDTAR

SEQ ID NO: 25235 - protein, 9 aa, synthetic construct
GGAGVDSLK

SEQ ID NO: 25236 - protein, 9 aa, synthetic construct
GGAGVDSLT

SEQ ID NO: 25237 - protein, 9 aa, synthetic construct
GGPGIDTLA

SEQ ID NO: 25238 - protein, 9 aa, synthetic construct
GGPGIDTAQ

SEQ ID NO: 25239 - protein, 9 aa, synthetic construct
GGAGVDSMS

SEQ ID NO: 25240 - protein, 9 aa, synthetic construct
GGAGVDSMV

SEQ ID NO: 25241 - protein, 9 aa, synthetic construct
GGGGDDQID

SEQ ID NO: 25242 - protein, 9 aa, synthetic construct
GGAGVDSMY

SEQ ID NO: 25243 - protein, 9 aa, synthetic construct
GGPGIDKLT

SEQ ID NO: 25244 - protein, 9 aa, synthetic construct
GGPGIDIAN

SEQ ID NO: 25245 - protein, 9 aa, synthetic construct
GGEGEDSLF

SEQ ID NO: 25246 - protein, 9 aa, synthetic construct
GGPGHDVMT

SEQ ID NO: 25247 - protein, 9 aa, synthetic construct
GGPGKDKLV

SEQ ID NO: 25248 - protein, 9 aa, synthetic construct
GGPGHDVLN

SEQ ID NO: 25249 - protein, 9 aa, synthetic construct
GGAGVDTFD

SEQ ID NO: 25250 - protein, 9 aa, synthetic construct
GGPGHDVIN

SEQ ID NO: 25251 - protein, 9 aa, synthetic construct
GGAGVDTFI

SEQ ID NO: 25252 - protein, 9 aa, synthetic construct
GGAGVDTFL

SEQ ID NO: 25253 - protein, 9 aa, synthetic construct
GGGGDDQLE

SEQ ID NO: 25254 - protein, 9 aa, synthetic construct
GGPGHDTLD

SEQ ID NO: 25255 - protein, 9 aa, synthetic construct
GGPGHDTIF

SEQ ID NO: 25256 - protein, 9 aa, synthetic construct
GGPGHDTIE

SEQ ID NO: 25257 - protein, 9 aa, synthetic construct
GGAGVDTIF

SEQ ID NO: 25258 - protein, 9 aa, synthetic construct
GGAGVDTIH

SEQ ID NO: 25259 - protein, 9 aa, synthetic construct
GGPGKDELV

SEQ ID NO: 25260 - protein, 9 aa, synthetic construct
GGAGVDSLA

SEQ ID NO: 25261 - protein, 9 aa, synthetic construct
GGPGNDAIW

SEQ ID NO: 25262 - protein, 9 aa, synthetic construct
GGPGLDLAS

SEQ ID NO: 25263 - protein, 9 aa, synthetic construct
GGAGVDRIH

SEQ ID NO: 25264 - protein, 9 aa, synthetic construct
GGAGVDRIL

SEQ ID NO: 25265 - protein, 9 aa, synthetic construct
GGEGEDTIY

SEQ ID NO: 25266 - protein, 9 aa, synthetic construct
GGGGDDNII

SEQ ID NO: 25267 - protein, 9 aa, synthetic construct
GGPGLDTLI

SEQ ID NO: 25268 - protein, 9 aa, synthetic construct
GGPGLDTLD

SEQ ID NO: 25269 - protein, 9 aa, synthetic construct
GGAGVDRLN

SEQ ID NO: 25270 - protein, 9 aa, synthetic construct
GGAGVDRLS

SEQ ID NO: 25271 - protein, 9 aa, synthetic construct
GGGGDDNIN

SEQ ID NO: 25272 - protein, 9 aa, synthetic construct
GGPGLDLLD

SEQ ID NO: 25273 - protein, 9 aa, synthetic construct
GGPGLDLIM

SEQ ID NO: 25274 - protein, 9 aa, synthetic construct
GGAGVDRMD

SEQ ID NO: 25275 - protein, 9 aa, synthetic construct
GGPGKDMFE

SEQ ID NO: 25276 - protein, 9 aa, synthetic construct
GGAGVDRMI

SEQ ID NO: 25277 - protein, 9 aa, synthetic construct
GGAGVDRMN

SEQ ID NO: 25278 - protein, 9 aa, synthetic construct
GGAGVDRVD

SEQ ID NO: 25279 - protein, 9 aa, synthetic construct
GGAGVDRVE

SEQ ID NO: 25280 - protein, 9 aa, synthetic construct
GGPGKDTLT

SEQ ID NO: 25281 - protein, 9 aa, synthetic construct
GGEGEDTIF

SEQ ID NO: 25282 - protein, 9 aa, synthetic construct
GGPGKDTLK

SEQ ID NO: 25283 - protein, 9 aa, synthetic construct
GGGGDDNLR

SEQ ID NO: 25284 - protein, 9 aa, synthetic construct
GGGGDDNLV

SEQ ID NO: 25285 - protein, 9 aa, synthetic construct
GGAGVDSIR

SEQ ID NO: 25286 - protein, 9 aa, synthetic construct
GGAGVDSIS

SEQ ID NO: 25287 - protein, 9 aa, synthetic construct
GGGGDDLMV

SEQ ID NO: 25288 - protein, 9 aa, synthetic construct
GGAGVDLLL

SEQ ID NO: 25289 - protein, 9 aa, synthetic construct
GGAGVDLLF

SEQ ID NO: 25290 - protein, 9 aa, synthetic construct
GGPGPDNLF

SEQ ID NO: 25291 - protein, 9 aa, synthetic construct
GGAGVDDMA

SEQ ID NO: 25292 - protein, 9 aa, synthetic construct
GGPGQDALY

SEQ ID NO: 25293 - protein, 9 aa, synthetic construct
GGEGEDVLS

SEQ ID NO: 25294 - protein, 9 aa, synthetic construct
GGGGDDKLA

SEQ ID NO: 25295 - protein, 9 aa, synthetic construct
GGPGPDTMT

SEQ ID NO: 25296 - protein, 9 aa, synthetic construct
GGAGVDELI

SEQ ID NO: 25297 - protein, 9 aa, synthetic construct
GGPGPDTLD

SEQ ID NO: 25298 - protein, 9 aa, synthetic construct
GGGGDDKLF

SEQ ID NO: 25299 - protein, 9 aa, synthetic construct
GGPGPDRLN

SEQ ID NO: 25300 - protein, 9 aa, synthetic construct
GGAGVDELY

SEQ ID NO: 25301 - protein, 9 aa, synthetic construct
GGPGPDQLK

SEQ ID NO: 25302 - protein, 9 aa, synthetic construct
GGEGEDVLQ

SEQ ID NO: 25303 - protein, 9 aa, synthetic construct
GGEGEDWID

SEQ ID NO: 25304 - protein, 9 aa, synthetic construct
GGPGPDLLI

SEQ ID NO: 25305 - protein, 9 aa, synthetic construct
GGAGVDFID

SEQ ID NO: 25306 - protein, 9 aa, synthetic construct
GGEGEDVLL

SEQ ID NO: 25307 - protein, 9 aa, synthetic construct
GGPGPDKFV

SEQ ID NO: 25308 - protein, 9 aa, synthetic construct
GGGGDDKLT

SEQ ID NO: 25309 - protein, 9 aa, synthetic construct
GGAGVDGLL

SEQ ID NO: 25310 - protein, 9 aa, synthetic construct
GGAGVDHFE

SEQ ID NO: 25311 - protein, 9 aa, synthetic construct
GGPGNDYLE

SEQ ID NO: 25312 - protein, 9 aa, synthetic construct
GGGGDDLFF

SEQ ID NO: 25313 - protein, 9 aa, synthetic construct
GGAGVDHFV

SEQ ID NO: 25314 - protein, 9 aa, synthetic construct
GGGGDDLFR

SEQ ID NO: 25315 - protein, 9 aa, synthetic construct
GGGGDDKIT

SEQ ID NO: 25316 - protein, 9 aa, synthetic construct
GGPGQDIAY

SEQ ID NO: 25317 - protein, 9 aa, synthetic construct
GGPGNDWID

SEQ ID NO: 25318 - protein, 9 aa, synthetic construct
GGPGQDRLR

SEQ ID NO: 25319 - protein, 9 aa, synthetic construct
GGPGRDCVS

SEQ ID NO: 25320 - protein, 9 aa, synthetic construct
GGAGTDYLQ

SEQ ID NO: 25321 - protein, 9 aa, synthetic construct
GGGGDDIVY

SEQ ID NO: 25322 - protein, 9 aa, synthetic construct
GGPGQDVAT

SEQ ID NO: 25323 - protein, 9 aa, synthetic construct
GGPGQDTLN

SEQ ID NO: 25324 - protein, 9 aa, synthetic construct
GGPGQDTLI

SEQ ID NO: 25325 - protein, 9 aa, synthetic construct
GGPGQDTLF

SEQ ID NO: 25326 - protein, 9 aa, synthetic construct
GGPGQDTLD

SEQ ID NO: 25327 - protein, 9 aa, synthetic construct
GGGGDDIYV

SEQ ID NO: 25328 - protein, 9 aa, synthetic construct
GGAGVDALN

SEQ ID NO: 25329 - protein, 9 aa, synthetic construct
GGAGVDALR

SEQ ID NO: 25330 - protein, 9 aa, synthetic construct
GGAGVDALT

SEQ ID NO: 25331 - protein, 9 aa, synthetic construct
GGPGQDILS

SEQ ID NO: 25332 - protein, 9 aa, synthetic construct
GGAGVDALV

SEQ ID NO: 25333 - protein, 9 aa, synthetic construct
GGAGVDALY

SEQ ID NO: 25334 - protein, 9 aa, synthetic construct
GGPGQDQLI

SEQ ID NO: 25335 - protein, 9 aa, synthetic construct
GGGGDDKAS

SEQ ID NO: 25336 - protein, 9 aa, synthetic construct
GGGGDDKID

SEQ ID NO: 25337 - protein, 9 aa, synthetic construct
GGPGQDMIN

SEQ ID NO: 25338 - protein, 9 aa, synthetic construct
GGPGQDLLT

SEQ ID NO: 25339 - protein, 9 aa, synthetic construct
GGPGQDLLH

SEQ ID NO: 25340 - protein, 9 aa, synthetic construct
GGGGDDKIF

SEQ ID NO: 25341 - protein, 9 aa, synthetic construct
GGEGEDWLY

SEQ ID NO: 25342 - protein, 9 aa, synthetic construct
GGPGQDILT

SEQ ID NO: 25343 - protein, 9 aa, synthetic construct
GGPGNDWLE

SEQ ID NO: 25344 - protein, 9 aa, synthetic construct
GGGGDDLFT

SEQ ID NO: 25345 - protein, 9 aa, synthetic construct
GGGGDDLMF

SEQ ID NO: 25346 - protein, 9 aa, synthetic construct
GGPGNDRLI

SEQ ID NO: 25347 - protein, 9 aa, synthetic construct
GGPGNDSIV

SEQ ID NO: 25348 - protein, 9 aa, synthetic construct
GGPGNDSIS

SEQ ID NO: 25349 - protein, 9 aa, synthetic construct
GGPGNDSIN

SEQ ID NO: 25350 - protein, 9 aa, synthetic construct
GGAGVDKIV

SEQ ID NO: 25351 - protein, 9 aa, synthetic construct
GGGGDDLLM

SEQ ID NO: 25352 - protein, 9 aa, synthetic construct
GGPGNDRYM

SEQ ID NO: 25353 - protein, 9 aa, synthetic construct
GGPGNDRYI

SEQ ID NO: 25354 - protein, 9 aa, synthetic construct
GGPGNDRVY

SEQ ID NO: 25355 - protein, 9 aa, synthetic construct
GGPGNDRMW

SEQ ID NO: 25356 - protein, 9 aa, synthetic construct
GGPGNDRLY

SEQ ID NO: 25357 - protein, 9 aa, synthetic construct
GGPGNDRLT

SEQ ID NO: 25358 - protein, 9 aa, synthetic construct
GGPGNDRLG

SEQ ID NO: 25359 - protein, 9 aa, synthetic construct
GGPGNDSVM

SEQ ID NO: 25360 - protein, 9 aa, synthetic construct
GGAGVDKMY

SEQ ID NO: 25361 - protein, 9 aa, synthetic construct
GGPGNDRIG

SEQ ID NO: 25362 - protein, 9 aa, synthetic construct
GGPGNDRIF

SEQ ID NO: 25363 - protein, 9 aa, synthetic construct
GGPGNDRID

SEQ ID NO: 25364 - protein, 9 aa, synthetic construct
GGAGVDLAS

SEQ ID NO: 25365 - protein, 9 aa, synthetic construct
GGEGEDTYL

SEQ ID NO: 25366 - protein, 9 aa, synthetic construct
GGPGNDQLR

SEQ ID NO: 25367 - protein, 9 aa, synthetic construct
GGPGNDQLH

SEQ ID NO: 25368 - protein, 9 aa, synthetic construct
GGAGVDLII

SEQ ID NO: 25369 - protein, 9 aa, synthetic construct
GGPGNDNMQ

SEQ ID NO: 25370 - protein, 9 aa, synthetic construct
GGGGDDLME

SEQ ID NO: 25371 - protein, 9 aa, synthetic construct
GGAGVDIVS

SEQ ID NO: 25372 - protein, 9 aa, synthetic construct
GGPGNDTAS

SEQ ID NO: 25373 - protein, 9 aa, synthetic construct
GGEGEDVIF

SEQ ID NO: 25374 - protein, 9 aa, synthetic construct
GGGGDDLIQ

SEQ ID NO: 25375 - protein, 9 aa, synthetic construct
GGPGNDVYN

SEQ ID NO: 25376 - protein, 9 aa, synthetic construct
GGPGNDVVD

SEQ ID NO: 25377 - protein, 9 aa, synthetic construct
GGPGNDVMT

SEQ ID NO: 25378 - protein, 9 aa, synthetic construct
GGPGNDVLW

SEQ ID NO: 25379 - protein, 9 aa, synthetic construct
GGGGDDLIL

SEQ ID NO: 25380 - protein, 9 aa, synthetic construct
GGPGNDVLQ

SEQ ID NO: 25381 - protein, 9 aa, synthetic construct
GGPGNDVLH

SEQ ID NO: 25382 - protein, 9 aa, synthetic construct
GGPGNDVLF

SEQ ID NO: 25383 - protein, 9 aa, synthetic construct
GGPGNDVLE

SEQ ID NO: 25384 - protein, 9 aa, synthetic construct
GGPGNDVIY

SEQ ID NO: 25385 - protein, 9 aa, synthetic construct
GGGGDDLIN

SEQ ID NO: 25386 - protein, 9 aa, synthetic construct
GGAGVDIID

SEQ ID NO: 25387 - protein, 9 aa, synthetic construct
GGPGNDTII

SEQ ID NO: 25388 - protein, 9 aa, synthetic construct
GGPGNDTYL

SEQ ID NO: 25389 - protein, 9 aa, synthetic construct
GGPGNDTVL

SEQ ID NO: 25390 - protein, 9 aa, synthetic construct
GGPGNDTVD

SEQ ID NO: 25391 - protein, 9 aa, synthetic construct
GGGGDDLIV

SEQ ID NO: 25392 - protein, 9 aa, synthetic construct
GGPGNDTMS

SEQ ID NO: 25393 - protein, 9 aa, synthetic construct
GGPGNDTMN

SEQ ID NO: 25394 - protein, 9 aa, synthetic construct
GGAGVDILI

SEQ ID NO: 25395 - protein, 9 aa, synthetic construct
GGAGVDILK

SEQ ID NO: 25396 - protein, 9 aa, synthetic construct
GGPGNDTIV

SEQ ID NO: 25397 - protein, 9 aa, synthetic construct
GGPGNDTIS

SEQ ID NO: 25398 - protein, 9 aa, synthetic construct
GGPGNDTIL

SEQ ID NO: 25399 - protein, 9 aa, synthetic construct
GGGGEDIFE

SEQ ID NO: 25400 - protein, 9 aa, synthetic construct
GGDGADQVQ

SEQ ID NO: 25401 - protein, 9 aa, synthetic construct
GGNGRDSLE

SEQ ID NO: 25402 - protein, 9 aa, synthetic construct
GGGGGDQMF

SEQ ID NO: 25403 - protein, 9 aa, synthetic construct
GGEGDDTAR

SEQ ID NO: 25404 - protein, 9 aa, synthetic construct
GGNGDDAVQ

SEQ ID NO: 25405 - protein, 9 aa, synthetic construct
GGNGDDAVD

SEQ ID NO: 25406 - protein, 9 aa, synthetic construct
GGDGDDRAW

SEQ ID NO: 25407 - protein, 9 aa, synthetic construct
GGNGDDALR

SEQ ID NO: 25408 - protein, 9 aa, synthetic construct
GGNGDDALQ

SEQ ID NO: 25409 - protein, 9 aa, synthetic construct
GGNGDDALH

SEQ ID NO: 25410 - protein, 9 aa, synthetic construct
GGDGDDRFE

SEQ ID NO: 25411 - protein, 9 aa, synthetic construct
GGNGDDAFH

SEQ ID NO: 25412 - protein, 9 aa, synthetic construct
GGNGCDRVW

SEQ ID NO: 25413 - protein, 9 aa, synthetic construct
GGDGDDRFV

SEQ ID NO: 25414 - protein, 9 aa, synthetic construct
GGDGDDRFW

SEQ ID NO: 25415 - protein, 9 aa, synthetic construct
GGDGDDRIH

SEQ ID NO: 25416 - protein, 9 aa, synthetic construct
GGNGADYLY

SEQ ID NO: 25417 - protein, 9 aa, synthetic construct
GGDGDDRIK

SEQ ID NO: 25418 - protein, 9 aa, synthetic construct
GGNGADYLD

SEQ ID NO: 25419 - protein, 9 aa, synthetic construct
GGDGDDRIN

SEQ ID NO: 25420 - protein, 9 aa, synthetic construct
GGGGGDRLT

SEQ ID NO: 25421 - protein, 9 aa, synthetic construct
GGNGADWMS

SEQ ID NO: 25422 - protein, 9 aa, synthetic construct
GGNGADWMN

SEQ ID NO: 25423 - protein, 9 aa, synthetic construct
GGNGADWLD

SEQ ID NO: 25424 - protein, 9 aa, synthetic construct
GGNGADVMR

SEQ ID NO: 25425 - protein, 9 aa, synthetic construct
GGNGADVLW

SEQ ID NO: 25426 - protein, 9 aa, synthetic construct
GGNGADVLQ

SEQ ID NO: 25427 - protein, 9 aa, synthetic construct
GGNGADVLF

SEQ ID NO: 25428 - protein, 9 aa, synthetic construct
GGDGDDQVL

SEQ ID NO: 25429 - protein, 9 aa, synthetic construct
GGNGDDDIQ

SEQ ID NO: 25430 - protein, 9 aa, synthetic construct
GGDGDDQMS

SEQ ID NO: 25431 - protein, 9 aa, synthetic construct
GGDGDDQIV

SEQ ID NO: 25432 - protein, 9 aa, synthetic construct
GGEGDDTFI

SEQ ID NO: 25433 - protein, 9 aa, synthetic construct
GGNGDDGLE

SEQ ID NO: 25434 - protein, 9 aa, synthetic construct
GGDGDDQIF

SEQ ID NO: 25435 - protein, 9 aa, synthetic construct
GGNGDDFVS

SEQ ID NO: 25436 - protein, 9 aa, synthetic construct
GGNGDDFVF

SEQ ID NO: 25437 - protein, 9 aa, synthetic construct
GGNGDDFMY

SEQ ID NO: 25438 - protein, 9 aa, synthetic construct
GGNGDDFLY

SEQ ID NO: 25439 - protein, 9 aa, synthetic construct
GGNGDDFLV

SEQ ID NO: 25440 - protein, 9 aa, synthetic construct
GGDGDDQII

SEQ ID NO: 25441 - protein, 9 aa, synthetic construct
GGNGDDFLD

SEQ ID NO: 25442 - protein, 9 aa, synthetic construct
GGDGDDQIT

SEQ ID NO: 25443 - protein, 9 aa, synthetic construct
GGGGGDRIH

SEQ ID NO: 25444 - protein, 9 aa, synthetic construct
GGDGDDQML

SEQ ID NO: 25445 - protein, 9 aa, synthetic construct
GGNGDDFIL

SEQ ID NO: 25446 - protein, 9 aa, synthetic construct
GGNGDDEVK

SEQ ID NO: 25447 - protein, 9 aa, synthetic construct
GGNGDDEVF

SEQ ID NO: 25448 - protein, 9 aa, synthetic construct
GGNGDDEMF

SEQ ID NO: 25449 - protein, 9 aa, synthetic construct
GGEGDDTFF

SEQ ID NO: 25450 - protein, 9 aa, synthetic construct
GGNGDDELV

SEQ ID NO: 25451 - protein, 9 aa, synthetic construct
GGNGDDELQ

SEQ ID NO: 25452 - protein, 9 aa, synthetic construct
GGNGDDELI

SEQ ID NO: 25453 - protein, 9 aa, synthetic construct
GGNGDDEIS

SEQ ID NO: 25454 - protein, 9 aa, synthetic construct
GGNGDDEFR

SEQ ID NO: 25455 - protein, 9 aa, synthetic construct
GGNGDDEFH

SEQ ID NO: 25456 - protein, 9 aa, synthetic construct
GGNGADVFF

SEQ ID NO: 25457 - protein, 9 aa, synthetic construct
GGGGGDRMI

SEQ ID NO: 25458 - protein, 9 aa, synthetic construct
GGNGADTVR

SEQ ID NO: 25459 - protein, 9 aa, synthetic construct
GGNGADNLT

SEQ ID NO: 25460 - protein, 9 aa, synthetic construct
GGNGADRIE

SEQ ID NO: 25461 - protein, 9 aa, synthetic construct
GGNGADQVL

SEQ ID NO: 25462 - protein, 9 aa, synthetic construct
GGNGADQLY

SEQ ID NO: 25463 - protein, 9 aa, synthetic construct
GGNGADQLV

SEQ ID NO: 25464 - protein, 9 aa, synthetic construct
GGNGADQLS

SEQ ID NO: 25465 - protein, 9 aa, synthetic construct
GGDGDDSME

SEQ ID NO: 25466 - protein, 9 aa, synthetic construct
GGEGDDSMV

SEQ ID NO: 25467 - protein, 9 aa, synthetic construct
GGGGGDSLD

SEQ ID NO: 25468 - protein, 9 aa, synthetic construct
GGNGADQIA

SEQ ID NO: 25469 - protein, 9 aa, synthetic construct
GGDGDDSMS

SEQ ID NO: 25470 - protein, 9 aa, synthetic construct
GGDGDDSMT

SEQ ID NO: 25471 - protein, 9 aa, synthetic construct
GGDGDDSMV

SEQ ID NO: 25472 - protein, 9 aa, synthetic construct
GGNGADRIV

SEQ ID NO: 25473 - protein, 9 aa, synthetic construct
GGNGADNLN

SEQ ID NO: 25474 - protein, 9 aa, synthetic construct
GGNGADNLD

SEQ ID NO: 25475 - protein, 9 aa, synthetic construct
GGNGADNIT

SEQ ID NO: 25476 - protein, 9 aa, synthetic construct
GGNGADNIS

SEQ ID NO: 25477 - protein, 9 aa, synthetic construct
GGDGDDSVE

SEQ ID NO: 25478 - protein, 9 aa, synthetic construct
GGNGADNID

SEQ ID NO: 25479 - protein, 9 aa, synthetic construct
GGNGADMIL

SEQ ID NO: 25480 - protein, 9 aa, synthetic construct
GGNGADMAS

SEQ ID NO: 25481 - protein, 9 aa, synthetic construct
GGDGDDSVW

SEQ ID NO: 25482 - protein, 9 aa, synthetic construct
GGDGDDSYI

SEQ ID NO: 25483 - protein, 9 aa, synthetic construct
GGNGADLLY

SEQ ID NO: 25484 - protein, 9 aa, synthetic construct
GGNGADRIN

SEQ ID NO: 25485 - protein, 9 aa, synthetic construct
GGNGADRIY

SEQ ID NO: 25486 - protein, 9 aa, synthetic construct
GGNGADTVN

SEQ ID NO: 25487 - protein, 9 aa, synthetic construct
GGDGDDRVY

SEQ ID NO: 25488 - protein, 9 aa, synthetic construct
GGDGDDRMY

SEQ ID NO: 25489 - protein, 9 aa, synthetic construct
GGDGDDRVF

SEQ ID NO: 25490 - protein, 9 aa, synthetic construct
GGGGGDRMK

SEQ ID NO: 25491 - protein, 9 aa, synthetic construct
GGNGADTML

SEQ ID NO: 25492 - protein, 9 aa, synthetic construct
GGNGADTMD

SEQ ID NO: 25493 - protein, 9 aa, synthetic construct
GGDGDDRVN

SEQ ID NO: 25494 - protein, 9 aa, synthetic construct
GGNGADTIT

SEQ ID NO: 25495 - protein, 9 aa, synthetic construct
GGNGADTIR

SEQ ID NO: 25496 - protein, 9 aa, synthetic construct
GGGGGDRYL

SEQ ID NO: 25497 - protein, 9 aa, synthetic construct
GGNGADTIL

SEQ ID NO: 25498 - protein, 9 aa, synthetic construct
GGNGADTIG

SEQ ID NO: 25499 - protein, 9 aa, synthetic construct
GGGGGDRYY

SEQ ID NO: 25500 - protein, 9 aa, synthetic construct
GGDGDDSLK

SEQ ID NO: 25501 - protein, 9 aa, synthetic construct
GGGGGDSFG

SEQ ID NO: 25502 - protein, 9 aa, synthetic construct
GGDGDDSAD

SEQ ID NO: 25503 - protein, 9 aa, synthetic construct
GGDGDDSAY

SEQ ID NO: 25504 - protein, 9 aa, synthetic construct
GGNGADSMS

SEQ ID NO: 25505 - protein, 9 aa, synthetic construct
GGNGADSMN

SEQ ID NO: 25506 - protein, 9 aa, synthetic construct
GGNGADSMA

SEQ ID NO: 25507 - protein, 9 aa, synthetic construct
GGNGADSLA

SEQ ID NO: 25508 - protein, 9 aa, synthetic construct
GGNGADSIT

SEQ ID NO: 25509 - protein, 9 aa, synthetic construct
GGNGADSIS

SEQ ID NO: 25510 - protein, 9 aa, synthetic construct
GGNGADSIL

SEQ ID NO: 25511 - protein, 9 aa, synthetic construct
GGDGDDSLH

SEQ ID NO: 25512 - protein, 9 aa, synthetic construct
GGNGDDGVY

SEQ ID NO: 25513 - protein, 9 aa, synthetic construct
GGGGGDQLY

SEQ ID NO: 25514 - protein, 9 aa, synthetic construct
GGDGADQVY

SEQ ID NO: 25515 - protein, 9 aa, synthetic construct
GGGGGDQLQ

SEQ ID NO: 25516 - protein, 9 aa, synthetic construct
GGNGDDTLQ

SEQ ID NO: 25517 - protein, 9 aa, synthetic construct
GGNGDDTIW

SEQ ID NO: 25518 - protein, 9 aa, synthetic construct
GGNGDDTIN

SEQ ID NO: 25519 - protein, 9 aa, synthetic construct
GGNGDDTII

SEQ ID NO: 25520 - protein, 9 aa, synthetic construct
GGNGDDTIA

SEQ ID NO: 25521 - protein, 9 aa, synthetic construct
GGNGDDTFY

SEQ ID NO: 25522 - protein, 9 aa, synthetic construct
GGNGDDTFR

SEQ ID NO: 25523 - protein, 9 aa, synthetic construct
GGNGDDTFF

SEQ ID NO: 25524 - protein, 9 aa, synthetic construct
GGNGDDSVT

SEQ ID NO: 25525 - protein, 9 aa, synthetic construct
GGNGDDSVF

SEQ ID NO: 25526 - protein, 9 aa, synthetic construct
GGNGDDSLL

SEQ ID NO: 25527 - protein, 9 aa, synthetic construct
GGNGDDSIX

SEQ ID NO: 25528 - protein, 9 aa, synthetic construct
GGNGDDSIL

SEQ ID NO: 25529 - protein, 9 aa, synthetic construct
GGDGDDLMD

SEQ ID NO: 25530 - protein, 9 aa, synthetic construct
GGNGDDRMS

SEQ ID NO: 25531 - protein, 9 aa, synthetic construct
GGGGGDLIK

SEQ ID NO: 25532 - protein, 9 aa, synthetic construct
GGDGDDLMN

SEQ ID NO: 25533 - protein, 9 aa, synthetic construct
GGNGDDRLV

SEQ ID NO: 25534 - protein, 9 aa, synthetic construct
GGNGDDRLR

SEQ ID NO: 25535 - protein, 9 aa, synthetic construct
GGNGDDRLI

SEQ ID NO: 25536 - protein, 9 aa, synthetic construct
GGNGDDRIY

SEQ ID NO: 25537 - protein, 9 aa, synthetic construct
GGDGDDLMS

SEQ ID NO: 25538 - protein, 9 aa, synthetic construct
GGNGDDRIE

SEQ ID NO: 25539 - protein, 9 aa, synthetic construct
GGNGDDRIA

SEQ ID NO: 25540 - protein, 9 aa, synthetic construct
GGNGDDRFV

SEQ ID NO: 25541 - protein, 9 aa, synthetic construct
GGDGDDLIQ

SEQ ID NO: 25542 - protein, 9 aa, synthetic construct
GGDGDDLIM

SEQ ID NO: 25543 - protein, 9 aa, synthetic construct
GGDGDDLIH

SEQ ID NO: 25544 - protein, 9 aa, synthetic construct
GGNGDDWID

SEQ ID NO: 25545 - protein, 9 aa, synthetic construct
GGNGDDYLV

SEQ ID NO: 25546 - protein, 9 aa, synthetic construct
GGNGDDYIQ

SEQ ID NO: 25547 - protein, 9 aa, synthetic construct
GGNGDDYIL

SEQ ID NO: 25548 - protein, 9 aa, synthetic construct
GGNGDDYIE

SEQ ID NO: 25549 - protein, 9 aa, synthetic construct
GGNGDDYIA

SEQ ID NO: 25550 - protein, 9 aa, synthetic construct
GGNGDDYFR

SEQ ID NO: 25551 - protein, 9 aa, synthetic construct
GGNGDDWMA

SEQ ID NO: 25552 - protein, 9 aa, synthetic construct
GGDGDDLAI

SEQ ID NO: 25553 - protein, 9 aa, synthetic construct
GGNGDDWLI

SEQ ID NO: 25554 - protein, 9 aa, synthetic construct
GGDGDDLAT

SEQ ID NO: 25555 - protein, 9 aa, synthetic construct
GGNGDDWIH

SEQ ID NO: 25556 - protein, 9 aa, synthetic construct
GGNGDDWIA

SEQ ID NO: 25557 - protein, 9 aa, synthetic construct
GGNGDDVAQ

SEQ ID NO: 25558 - protein, 9 aa, synthetic construct
GGNGDDWAS

SEQ ID NO: 25559 - protein, 9 aa, synthetic construct
GGNGDDVVI

SEQ ID NO: 25560 - protein, 9 aa, synthetic construct
GGNGDDVMY

SEQ ID NO: 25561 - protein, 9 aa, synthetic construct
GGNGDDVMF

SEQ ID NO: 25562 - protein, 9 aa, synthetic construct
GGNGDDVLC

SEQ ID NO: 25563 - protein, 9 aa, synthetic construct
GGNGDDVIW

SEQ ID NO: 25564 - protein, 9 aa, synthetic construct
GGNGDDVIR

SEQ ID NO: 25565 - protein, 9 aa, synthetic construct
GGNGDDVIL

SEQ ID NO: 25566 - protein, 9 aa, synthetic construct
GGNGDDVIH

SEQ ID NO: 25567 - protein, 9 aa, synthetic construct
GGNGDDVIE

SEQ ID NO: 25568 - protein, 9 aa, synthetic construct
GGNGDDVID

SEQ ID NO: 25569 - protein, 9 aa, synthetic construct
GGGGGDLLF

SEQ ID NO: 25570 - protein, 9 aa, synthetic construct
GGDGDDLVF

SEQ ID NO: 25571 - protein, 9 aa, synthetic construct
GGNGDDQLN

SEQ ID NO: 25572 - protein, 9 aa, synthetic construct
GGNGDDIMY

SEQ ID NO: 25573 - protein, 9 aa, synthetic construct
GGDGDDMLM

SEQ ID NO: 25574 - protein, 9 aa, synthetic construct
GGNGDDLAN

SEQ ID NO: 25575 - protein, 9 aa, synthetic construct
GGNGDDKLQ

SEQ ID NO: 25576 - protein, 9 aa, synthetic construct
GGNGDDKLN

SEQ ID NO: 25577 - protein, 9 aa, synthetic construct
GGNGDDKLI

SEQ ID NO: 25578 - protein, 9 aa, synthetic construct
GGEGDDTIR

SEQ ID NO: 25579 - protein, 9 aa, synthetic construct
GGNGDDKIW

SEQ ID NO: 25580 - protein, 9 aa, synthetic construct
GGDGDDNII

SEQ ID NO: 25581 - protein, 9 aa, synthetic construct
GGDGDDNIR

SEQ ID NO: 25582 - protein, 9 aa, synthetic construct
GGDGDDNLA

SEQ ID NO: 25583 - protein, 9 aa, synthetic construct
GGDGDDNLE

SEQ ID NO: 25584 - protein, 9 aa, synthetic construct
GGNGDDIMD

SEQ ID NO: 25585 - protein, 9 aa, synthetic construct
GGGGGDLMY

SEQ ID NO: 25586 - protein, 9 aa, synthetic construct
GGNGDDILT

SEQ ID NO: 25587 - protein, 9 aa, synthetic construct
GGNGDDILS

SEQ ID NO: 25588 - protein, 9 aa, synthetic construct
GGNGDDILK

SEQ ID NO: 25589 - protein, 9 aa, synthetic construct
GGNGDDILG

SEQ ID NO: 25590 - protein, 9 aa, synthetic construct
GGEGDDTIE

SEQ ID NO: 25591 - protein, 9 aa, synthetic construct
GGNGDDIIR

SEQ ID NO: 25592 - protein, 9 aa, synthetic construct
GGNGDDIII

SEQ ID NO: 25593 - protein, 9 aa, synthetic construct
GGDGDDNLV

SEQ ID NO: 25594 - protein, 9 aa, synthetic construct
GGNGDDIAL

SEQ ID NO: 25595 - protein, 9 aa, synthetic construct
GGEGDDTIA

SEQ ID NO: 25596 - protein, 9 aa, synthetic construct
GGNGDDHLV

SEQ ID NO: 25597 - protein, 9 aa, synthetic construct
GGNGDDLIE

SEQ ID NO: 25598 - protein, 9 aa, synthetic construct
GGNGDDLIT

SEQ ID NO: 25599 - protein, 9 aa, synthetic construct
GGNGDDQLI

SEQ ID NO: 25600 - protein, 9 aa, synthetic construct
GGNGDDMVR

SEQ ID NO: 25601 - protein, 9 aa, synthetic construct
GGNGDDQLH

SEQ ID NO: 25602 - protein, 9 aa, synthetic construct
GGNGDDQLD

SEQ ID NO: 25603 - protein, 9 aa, synthetic construct
GGNGDDQLA

SEQ ID NO: 25604 - protein, 9 aa, synthetic construct
GGNGDDQIG

SEQ ID NO: 25605 - protein, 9 aa, synthetic construct
GGDGDDLVV

SEQ ID NO: 25606 - protein, 9 aa, synthetic construct
GGDGDDLVW

SEQ ID NO: 25607 - protein, 9 aa, synthetic construct
GGDGDDLYI

SEQ ID NO: 25608 - protein, 9 aa, synthetic construct
GGDGDDLYL

SEQ ID NO: 25609 - protein, 9 aa, synthetic construct
GGNGDDNLY

SEQ ID NO: 25610 - protein, 9 aa, synthetic construct
GGNGDDNLT

SEQ ID NO: 25611 - protein, 9 aa, synthetic construct
GGDGDDLYQ

SEQ ID NO: 25612 - protein, 9 aa, synthetic construct
GGNGDDMLY

SEQ ID NO: 25613 - protein, 9 aa, synthetic construct
GGNGDDLLM

SEQ ID NO: 25614 - protein, 9 aa, synthetic construct
GGNGDDMLS

SEQ ID NO: 25615 - protein, 9 aa, synthetic construct
GGDGDDMIF

SEQ ID NO: 25616 - protein, 9 aa, synthetic construct
GGDGDDMIV

SEQ ID NO: 25617 - protein, 9 aa, synthetic construct
GGNGDDMIG

SEQ ID NO: 25618 - protein, 9 aa, synthetic construct
GGDGDDMIY

SEQ ID NO: 25619 - protein, 9 aa, synthetic construct
GGNGDDMFH

SEQ ID NO: 25620 - protein, 9 aa, synthetic construct
GGNGDDLVV

SEQ ID NO: 25621 - protein, 9 aa, synthetic construct
GGNGDDLVS

SEQ ID NO: 25622 - protein, 9 aa, synthetic construct
GGNGDDLMS

SEQ ID NO: 25623 - protein, 9 aa, synthetic construct
GGDGDDMLE

SEQ ID NO: 25624 - protein, 9 aa, synthetic construct
GGNGDDLLN

SEQ ID NO: 25625 - protein, 9 aa, synthetic construct
GGNGADLLV

SEQ ID NO: 25626 - protein, 9 aa, synthetic construct
GGNGADLLR

SEQ ID NO: 25627 - protein, 9 aa, synthetic construct
GGNGADLLF

SEQ ID NO: 25628 - protein, 9 aa, synthetic construct
GGNGADLIY

SEQ ID NO: 25629 - protein, 9 aa, synthetic construct
GGEGDDSIV

SEQ ID NO: 25630 - protein, 9 aa, synthetic construct
GGGGGDVID

SEQ ID NO: 25631 - protein, 9 aa, synthetic construct
GGDGEDEFV

SEQ ID NO: 25632 - protein, 9 aa, synthetic construct
GGMGEDVLY

SEQ ID NO: 25633 - protein, 9 aa, synthetic construct
GGDGEDEID

SEQ ID NO: 25634 - protein, 9 aa, synthetic construct
GGGGGDVIT

SEQ ID NO: 25635 - protein, 9 aa, synthetic construct
GGMGEDTLI

SEQ ID NO: 25636 - protein, 9 aa, synthetic construct
GGGGGDVLA

SEQ ID NO: 25637 - protein, 9 aa, synthetic construct
GGDGEDELF

SEQ ID NO: 25638 - protein, 9 aa, synthetic construct
GGDGEDELL

SEQ ID NO: 25639 - protein, 9 aa, synthetic construct
GGMGEDMLD

SEQ ID NO: 25640 - protein, 9 aa, synthetic construct
GGEGDDSIN

SEQ ID NO: 25641 - protein, 9 aa, synthetic construct
GGDGEDFIN

SEQ ID NO: 25642 - protein, 9 aa, synthetic construct
GGGGGDVLQ

SEQ ID NO: 25643 - protein, 9 aa, synthetic construct
GGDGEDFLL

SEQ ID NO: 25644 - protein, 9 aa, synthetic construct
GGDGEDFLS

SEQ ID NO: 25645 - protein, 9 aa, synthetic construct
GGMGDDYIE

SEQ ID NO: 25646 - protein, 9 aa, synthetic construct
GGDGEDFVN

SEQ ID NO: 25647 - protein, 9 aa, synthetic construct
GGMGDDWLE

SEQ ID NO: 25648 - protein, 9 aa, synthetic construct
GGEGDDSII

SEQ ID NO: 25649 - protein, 9 aa, synthetic construct
GGGGGDVLT

SEQ ID NO: 25650 - protein, 9 aa, synthetic construct
GGGGGDVLY

SEQ ID NO: 25651 - protein, 9 aa, synthetic construct
GGDGEDHAF

SEQ ID NO: 25652 - protein, 9 aa, synthetic construct
GGDGEDHLE

SEQ ID NO: 25653 - protein, 9 aa, synthetic construct
GGMGDDVLL

SEQ ID NO: 25654 - protein, 9 aa, synthetic construct
GGGGGDVFV

SEQ ID NO: 25655 - protein, 9 aa, synthetic construct
GGDGEDDIY

SEQ ID NO: 25656 - protein, 9 aa, synthetic construct
GGMGGDILT

SEQ ID NO: 25657 - protein, 9 aa, synthetic construct
GGDGDDYLM

SEQ ID NO: 25658 - protein, 9 aa, synthetic construct
GGDGDDYAD

SEQ ID NO: 25659 - protein, 9 aa, synthetic construct
GGMGNDFLD

SEQ ID NO: 25660 - protein, 9 aa, synthetic construct
GGDGDDYFE

SEQ ID NO: 25661 - protein, 9 aa, synthetic construct
GGMGNDDLL

SEQ ID NO: 25662 - protein, 9 aa, synthetic construct
GGMGMDTLD

SEQ ID NO: 25663 - protein, 9 aa, synthetic construct
GGMGLDIAD

SEQ ID NO: 25664 - protein, 9 aa, synthetic construct
GGMGLDHLT

SEQ ID NO: 25665 - protein, 9 aa, synthetic construct
GGGGGDTVN

SEQ ID NO: 25666 - protein, 9 aa, synthetic construct
GGMGKDQLT

SEQ ID NO: 25667 - protein, 9 aa, synthetic construct
GGMGKDILT

SEQ ID NO: 25668 - protein, 9 aa, synthetic construct
GGGGGDTVV

SEQ ID NO: 25669 - protein, 9 aa, synthetic construct
GGGGGDTYL

SEQ ID NO: 25670 - protein, 9 aa, synthetic construct
GGDGEDAVY

SEQ ID NO: 25671 - protein, 9 aa, synthetic construct
GGDGDDYMD

SEQ ID NO: 25672 - protein, 9 aa, synthetic construct
GGDGDDYMV

SEQ ID NO: 25673 - protein, 9 aa, synthetic construct
GGGGGDTYV

SEQ ID NO: 25674 - protein, 9 aa, synthetic construct
GGMGHDIVS

SEQ ID NO: 25675 - protein, 9 aa, synthetic construct
GGGGGDTYY

SEQ ID NO: 25676 - protein, 9 aa, synthetic construct
GGMGGDVLL

SEQ ID NO: 25677 - protein, 9 aa, synthetic construct
GGMGGDVFV

SEQ ID NO: 25678 - protein, 9 aa, synthetic construct
GGDGDDYVN

SEQ ID NO: 25679 - protein, 9 aa, synthetic construct
GGDGDDYVS

SEQ ID NO: 25680 - protein, 9 aa, synthetic construct
GGDGEDALT

SEQ ID NO: 25681 - protein, 9 aa, synthetic construct
GGMGGDLLT

SEQ ID NO: 25682 - protein, 9 aa, synthetic construct
GGGGGDVMN

SEQ ID NO: 25683 - protein, 9 aa, synthetic construct
GGEGDDSIF

SEQ ID NO: 25684 - protein, 9 aa, synthetic construct
GGDGEDILV

SEQ ID NO: 25685 - protein, 9 aa, synthetic construct
GGDGEDSID

SEQ ID NO: 25686 - protein, 9 aa, synthetic construct
GGEGDDRMH

SEQ ID NO: 25687 - protein, 9 aa, synthetic construct
GGMGDDFIN

SEQ ID NO: 25688 - protein, 9 aa, synthetic construct
GGMGDDFID

SEQ ID NO: 25689 - protein, 9 aa, synthetic construct
GGDGEDRLI

SEQ ID NO: 25690 - protein, 9 aa, synthetic construct
GGEGDDRMF

SEQ ID NO: 25691 - protein, 9 aa, synthetic construct
GGMGDDALY

SEQ ID NO: 25692 - protein, 9 aa, synthetic construct
GGMGDDALS

SEQ ID NO: 25693 - protein, 9 aa, synthetic construct
GGDGEDRLV

SEQ ID NO: 25694 - protein, 9 aa, synthetic construct
GGGGHDEIY

SEQ ID NO: 25695 - protein, 9 aa, synthetic construct
GGMGADVLV

SEQ ID NO: 25696 - protein, 9 aa, synthetic construct
GGEGDDRLW

SEQ ID NO: 25697 - protein, 9 aa, synthetic construct
GGMGADVLH

SEQ ID NO: 25698 - protein, 9 aa, synthetic construct
GGMGDDIFV

SEQ ID NO: 25699 - protein, 9 aa, synthetic construct
GGMGADVFV

SEQ ID NO: 25700 - protein, 9 aa, synthetic construct
GGMGADVFQ

SEQ ID NO: 25701 - protein, 9 aa, synthetic construct
GGGGHDELT

SEQ ID NO: 25702 - protein, 9 aa, synthetic construct
GGMGADTMD

SEQ ID NO: 25703 - protein, 9 aa, synthetic construct
GGMGADTLQ

SEQ ID NO: 25704 - protein, 9 aa, synthetic construct
GGDGEDSLF

SEQ ID NO: 25705 - protein, 9 aa, synthetic construct
GGMGADTFL

SEQ ID NO: 25706 - protein, 9 aa, synthetic construct
GGMGADSVY

SEQ ID NO: 25707 - protein, 9 aa, synthetic construct
GGMGADSLS

SEQ ID NO: 25708 - protein, 9 aa, synthetic construct
GGMGADSID

SEQ ID NO: 25709 - protein, 9 aa, synthetic construct
GGMGADRMR

SEQ ID NO: 25710 - protein, 9 aa, synthetic construct
GGMGDDHLR

SEQ ID NO: 25711 - protein, 9 aa, synthetic construct
GGDGEDRLF

SEQ ID NO: 25712 - protein, 9 aa, synthetic construct
GGGGGDVYL

SEQ ID NO: 25713 - protein, 9 aa, synthetic construct
GGEGDDRYF

SEQ ID NO: 25714 - protein, 9 aa, synthetic construct
GGMGDDTLI

SEQ ID NO: 25715 - protein, 9 aa, synthetic construct
GGGGGDWLS

SEQ ID NO: 25716 - protein, 9 aa, synthetic construct
GGMGDDTID

SEQ ID NO: 25717 - protein, 9 aa, synthetic construct
GGGGGDWVV

SEQ ID NO: 25718 - protein, 9 aa, synthetic construct
GGMGDDSML

SEQ ID NO: 25719 - protein, 9 aa, synthetic construct
GGGGGDYIY

SEQ ID NO: 25720 - protein, 9 aa, synthetic construct
GGDGEDLLR

SEQ ID NO: 25721 - protein, 9 aa, synthetic construct
GGDGEDLLS

SEQ ID NO: 25722 - protein, 9 aa, synthetic construct
GGGGGDYLQ

SEQ ID NO: 25723 - protein, 9 aa, synthetic construct
GGDGEDMLV

SEQ ID NO: 25724 - protein, 9 aa, synthetic construct
GGDGEDNLS

SEQ ID NO: 25725 - protein, 9 aa, synthetic construct
GGMGDDMLL

SEQ ID NO: 25726 - protein, 9 aa, synthetic construct
GGMGDDIIN

SEQ ID NO: 25727 - protein, 9 aa, synthetic construct
GGDGEDQLS

SEQ ID NO: 25728 - protein, 9 aa, synthetic construct
GGGGHDALD

SEQ ID NO: 25729 - protein, 9 aa, synthetic construct
GGMGDDLLL

SEQ ID NO: 25730 - protein, 9 aa, synthetic construct
GGMGDDLLA

SEQ ID NO: 25731 - protein, 9 aa, synthetic construct
GGMGDDLII

SEQ ID NO: 25732 - protein, 9 aa, synthetic construct
GGMGDDLIF

SEQ ID NO: 25733 - protein, 9 aa, synthetic construct
GGEGDDRVD

SEQ ID NO: 25734 - protein, 9 aa, synthetic construct
GGGGHDDLD

SEQ ID NO: 25735 - protein, 9 aa, synthetic construct
GGMGDDILQ

SEQ ID NO: 25736 - protein, 9 aa, synthetic construct
GGMGDDILF

SEQ ID NO: 25737 - protein, 9 aa, synthetic construct
GGEGDDRMS

SEQ ID NO: 25738 - protein, 9 aa, synthetic construct
GGMGNDFLV

SEQ ID NO: 25739 - protein, 9 aa, synthetic construct
GGMGNDFLY

SEQ ID NO: 25740 - protein, 9 aa, synthetic construct
GGMGNDFVV

SEQ ID NO: 25741 - protein, 9 aa, synthetic construct
GGMGTDLLN

SEQ ID NO: 25742 - protein, 9 aa, synthetic construct
GGGGGDSVE

SEQ ID NO: 25743 - protein, 9 aa, synthetic construct
GGMGVDTLY

SEQ ID NO: 25744 - protein, 9 aa, synthetic construct
GGGGGDSYL

SEQ ID NO: 25745 - protein, 9 aa, synthetic construct
GGMGVDTLI

SEQ ID NO: 25746 - protein, 9 aa, synthetic construct
GGMGVDTLD

SEQ ID NO: 25747 - protein, 9 aa, synthetic construct
GGMGVDSLD

SEQ ID NO: 25748 - protein, 9 aa, synthetic construct
GGDGDDTMS

SEQ ID NO: 25749 - protein, 9 aa, synthetic construct
GGMGTDTLI

SEQ ID NO: 25750 - protein, 9 aa, synthetic construct
GGDGDDTMY

SEQ ID NO: 25751 - protein, 9 aa, synthetic construct
GGDGDDTVA

SEQ ID NO: 25752 - protein, 9 aa, synthetic construct
GGMGTDNLT

SEQ ID NO: 25753 - protein, 9 aa, synthetic construct
GGMGTDILT

SEQ ID NO: 25754 - protein, 9 aa, synthetic construct
GGDGDDTMD

SEQ ID NO: 25755 - protein, 9 aa, synthetic construct
GGMGTDELI

SEQ ID NO: 25756 - protein, 9 aa, synthetic construct
GGMGSDVYL

SEQ ID NO: 25757 - protein, 9 aa, synthetic construct
GGMGSDVLR

SEQ ID NO: 25758 - protein, 9 aa, synthetic construct
GGDGDDTVN

SEQ ID NO: 25759 - protein, 9 aa, synthetic construct
GGMGSDTLS

SEQ ID NO: 25760 - protein, 9 aa, synthetic construct
GGDGDDTVW

SEQ ID NO: 25761 - protein, 9 aa, synthetic construct
GGDGDDTYA

SEQ ID NO: 25762 - protein, 9 aa, synthetic construct
GGMGSDRLF

SEQ ID NO: 25763 - protein, 9 aa, synthetic construct
GGDGDDTYE

SEQ ID NO: 25764 - protein, 9 aa, synthetic construct
GGMGSDILN

SEQ ID NO: 25765 - protein, 9 aa, synthetic construct
GGMGSDILA

SEQ ID NO: 25766 - protein, 9 aa, synthetic construct
GGMGVDTMI

SEQ ID NO: 25767 - protein, 9 aa, synthetic construct
GGNGADAIF

SEQ ID NO: 25768 - protein, 9 aa, synthetic construct
GGGGGDTFQ

SEQ ID NO: 25769 - protein, 9 aa, synthetic construct
GGNGADILY

SEQ ID NO: 25770 - protein, 9 aa, synthetic construct
GGDGDDTAI

SEQ ID NO: 25771 - protein, 9 aa, synthetic construct
GGGGGDSLS

SEQ ID NO: 25772 - protein, 9 aa, synthetic construct
GGDGDDTAS

SEQ ID NO: 25773 - protein, 9 aa, synthetic construct
GGDGDDTAV

SEQ ID NO: 25774 - protein, 9 aa, synthetic construct
GGDGDDTAY

SEQ ID NO: 25775 - protein, 9 aa, synthetic construct
GGNGADKLE

SEQ ID NO: 25776 - protein, 9 aa, synthetic construct
GGDGDDTFN

SEQ ID NO: 25777 - protein, 9 aa, synthetic construct
GGNGADKID

SEQ ID NO: 25778 - protein, 9 aa, synthetic construct
GGGGGDSLY

SEQ ID NO: 25779 - protein, 9 aa, synthetic construct
GGNGADIVD

SEQ ID NO: 25780 - protein, 9 aa, synthetic construct
GGNGADIMD

SEQ ID NO: 25781 - protein, 9 aa, synthetic construct
GGNGADILI

SEQ ID NO: 25782 - protein, 9 aa, synthetic construct
GGNGADALF

SEQ ID NO: 25783 - protein, 9 aa, synthetic construct
GGNGADILA

SEQ ID NO: 25784 - protein, 9 aa, synthetic construct
GGNGADIIY

SEQ ID NO: 25785 - protein, 9 aa, synthetic construct
GGNGADIIG

SEQ ID NO: 25786 - protein, 9 aa, synthetic construct
GGNGADIID

SEQ ID NO: 25787 - protein, 9 aa, synthetic construct
GGNGADIFV

SEQ ID NO: 25788 - protein, 9 aa, synthetic construct
GGNGADHLD

SEQ ID NO: 25789 - protein, 9 aa, synthetic construct
GGNGADFLY

SEQ ID NO: 25790 - protein, 9 aa, synthetic construct
GGNGADFLV

SEQ ID NO: 25791 - protein, 9 aa, synthetic construct
GGNGADELS

SEQ ID NO: 25792 - protein, 9 aa, synthetic construct
GGNGADELN

SEQ ID NO: 25793 - protein, 9 aa, synthetic construct
GGNGADDLR

SEQ ID NO: 25794 - protein, 9 aa, synthetic construct
GGDGDDTYM

SEQ ID NO: 25795 - protein, 9 aa, synthetic construct
GGMGSDHLT

SEQ ID NO: 25796 - protein, 9 aa, synthetic construct
GGDGDDWMK

SEQ ID NO: 25797 - protein, 9 aa, synthetic construct
GGMGNDRLM

SEQ ID NO: 25798 - protein, 9 aa, synthetic construct
GGMGNDTLW

SEQ ID NO: 25799 - protein, 9 aa, synthetic construct
GGDGDDVVD

SEQ ID NO: 25800 - protein, 9 aa, synthetic construct
GGMGNDTLA

SEQ ID NO: 25801 - protein, 9 aa, synthetic construct
GGDGDDVVH

SEQ ID NO: 25802 - protein, 9 aa, synthetic construct
GGMGNDTIN

SEQ ID NO: 25803 - protein, 9 aa, synthetic construct
GGMGNDTIL

SEQ ID NO: 25804 - protein, 9 aa, synthetic construct
GGMGNDTIA

SEQ ID NO: 25805 - protein, 9 aa, synthetic construct
GGMGNDTAY

SEQ ID NO: 25806 - protein, 9 aa, synthetic construct
GGMGNDSLS

SEQ ID NO: 25807 - protein, 9 aa, synthetic construct
GGMGNDSLL

SEQ ID NO: 25808 - protein, 9 aa, synthetic construct
GGMGNDSIT

SEQ ID NO: 25809 - protein, 9 aa, synthetic construct
GGDGDDWFD

SEQ ID NO: 25810 - protein, 9 aa, synthetic construct
GGMGNDTMI

SEQ ID NO: 25811 - protein, 9 aa, synthetic construct
GGMGNDQLR

SEQ ID NO: 25812 - protein, 9 aa, synthetic construct
GGGGGDTLK

SEQ ID NO: 25813 - protein, 9 aa, synthetic construct
GGMGNDMIN

SEQ ID NO: 25814 - protein, 9 aa, synthetic construct
GGDGDDWIQ

SEQ ID NO: 25815 - protein, 9 aa, synthetic construct
GGMGNDLIY

SEQ ID NO: 25816 - protein, 9 aa, synthetic construct
GGMGNDKMN

SEQ ID NO: 25817 - protein, 9 aa, synthetic construct
GGMGNDKMD

SEQ ID NO: 25818 - protein, 9 aa, synthetic construct
GGMGNDKLF

SEQ ID NO: 25819 - protein, 9 aa, synthetic construct
GGMGNDIYY

SEQ ID NO: 25820 - protein, 9 aa, synthetic construct
GGDGDDWLR

SEQ ID NO: 25821 - protein, 9 aa, synthetic construct
GGMGNDILY

SEQ ID NO: 25822 - protein, 9 aa, synthetic construct
GGDGDDVMY

SEQ ID NO: 25823 - protein, 9 aa, synthetic construct
GGMGNDTMS

SEQ ID NO: 25824 - protein, 9 aa, synthetic construct
GGDGDDVAV

SEQ ID NO: 25825 - protein, 9 aa, synthetic construct
GGGGGDTID

SEQ ID NO: 25826 - protein, 9 aa, synthetic construct
GGMGRDVMT

SEQ ID NO: 25827 - protein, 9 aa, synthetic construct
GGDGDDVAY

SEQ ID NO: 25828 - protein, 9 aa, synthetic construct
GGDGDDVFA

SEQ ID NO: 25829 - protein, 9 aa, synthetic construct
GGMGRDVLH

SEQ ID NO: 25830 - protein, 9 aa, synthetic construct
GGDGDDVFF

SEQ ID NO: 25831 - protein, 9 aa, synthetic construct
GGDGDDVFI

SEQ ID NO: 25832 - protein, 9 aa, synthetic construct
GGMGRDTYY

SEQ ID NO: 25833 - protein, 9 aa, synthetic construct
GGMGRDTVD

SEQ ID NO: 25834 - protein, 9 aa, synthetic construct
GGMGRDTLN

SEQ ID NO: 25835 - protein, 9 aa, synthetic construct
GGMGRDTIS

SEQ ID NO: 25836 - protein, 9 aa, synthetic construct
GGMGRDMLN

SEQ ID NO: 25837 - protein, 9 aa, synthetic construct
GGMGQDVML

SEQ ID NO: 25838 - protein, 9 aa, synthetic construct
GGEGDDSLQ

SEQ ID NO: 25839 - protein, 9 aa, synthetic construct
GGMGQDTMT

SEQ ID NO: 25840 - protein, 9 aa, synthetic construct
GGMGQDTLW

SEQ ID NO: 25841 - protein, 9 aa, synthetic construct
GGMGQDTLF

SEQ ID NO: 25842 - protein, 9 aa, synthetic construct
GGMGQDIMT

SEQ ID NO: 25843 - protein, 9 aa, synthetic construct
GGMGNDWMH

SEQ ID NO: 25844 - protein, 9 aa, synthetic construct
GGMGNDVLR

SEQ ID NO: 25845 - protein, 9 aa, synthetic construct
GGMGNDVLI

SEQ ID NO: 25846 - protein, 9 aa, synthetic construct
GGMGNDVFV

SEQ ID NO: 25847 - protein, 9 aa, synthetic construct
GGDGDDVMG

SEQ ID NO: 25848 - protein, 9 aa, synthetic construct
GGDGDDVMI

SEQ ID NO: 25849 - protein, 9 aa, synthetic construct
GGGGGDTIE

SEQ ID NO: 25850 - protein, 9 aa, synthetic construct
GGDGDDKMA

SEQ ID NO: 25851 - protein, 9 aa, synthetic construct
GGNGDDYVL

SEQ ID NO: 25852 - protein, 9 aa, synthetic construct
GGNGDDYYV

SEQ ID NO: 25853 - protein, 9 aa, synthetic construct
GGGGFDELF

SEQ ID NO: 25854 - protein, 9 aa, synthetic construct
GGDGADVII

SEQ ID NO: 25855 - protein, 9 aa, synthetic construct
GGNGNDQID

SEQ ID NO: 25856 - protein, 9 aa, synthetic construct
GGNGNDNVQ

SEQ ID NO: 25857 - protein, 9 aa, synthetic construct
GGDGADVIR

SEQ ID NO: 25858 - protein, 9 aa, synthetic construct
GGDGADVIS

SEQ ID NO: 25859 - protein, 9 aa, synthetic construct
GGNGNDNLH

SEQ ID NO: 25860 - protein, 9 aa, synthetic construct
GGNGNDNLD

SEQ ID NO: 25861 - protein, 9 aa, synthetic construct
GGNGNDMLT

SEQ ID NO: 25862 - protein, 9 aa, synthetic construct
GGNGNDMLN

SEQ ID NO: 25863 - protein, 9 aa, synthetic construct
GGDGADVLG

SEQ ID NO: 25864 - protein, 9 aa, synthetic construct
GGNGNDMLE

SEQ ID NO: 25865 - protein, 9 aa, synthetic construct
GGNGNDMLA

SEQ ID NO: 25866 - protein, 9 aa, synthetic construct
GGNGNDLVN

SEQ ID NO: 25867 - protein, 9 aa, synthetic construct
GGNGNDLVG

SEQ ID NO: 25868 - protein, 9 aa, synthetic construct
GGNGNDLMI

SEQ ID NO: 25869 - protein, 9 aa, synthetic construct
GGNGNDLIT

SEQ ID NO: 25870 - protein, 9 aa, synthetic construct
GGNGNDLIQ

SEQ ID NO: 25871 - protein, 9 aa, synthetic construct
GGNGNDLIK

SEQ ID NO: 25872 - protein, 9 aa, synthetic construct
GGGGEDTIM

SEQ ID NO: 25873 - protein, 9 aa, synthetic construct
GGDGADVMF

SEQ ID NO: 25874 - protein, 9 aa, synthetic construct
GGDGADVMH

SEQ ID NO: 25875 - protein, 9 aa, synthetic construct
GGDGADVMR

SEQ ID NO: 25876 - protein, 9 aa, synthetic construct
GGNGNDLAY

SEQ ID NO: 25877 - protein, 9 aa, synthetic construct
GGDGADVMT

SEQ ID NO: 25878 - protein, 9 aa, synthetic construct
GGGGEDTIY

SEQ ID NO: 25879 - protein, 9 aa, synthetic construct
GGNGNDQLE

SEQ ID NO: 25880 - protein, 9 aa, synthetic construct
GGNGNDQLM

SEQ ID NO: 25881 - protein, 9 aa, synthetic construct
GGNGNDQLS

SEQ ID NO: 25882 - protein, 9 aa, synthetic construct
GGDGADTYL

SEQ ID NO: 25883 - protein, 9 aa, synthetic construct
GGNGNDSYT

SEQ ID NO: 25884 - protein, 9 aa, synthetic construct
GGDGADTMV

SEQ ID NO: 25885 - protein, 9 aa, synthetic construct
GGDGADTVA

SEQ ID NO: 25886 - protein, 9 aa, synthetic construct
GGDGADTVD

SEQ ID NO: 25887 - protein, 9 aa, synthetic construct
GGNGNDSMQ

SEQ ID NO: 25888 - protein, 9 aa, synthetic construct
GGNGNDSLM

SEQ ID NO: 25889 - protein, 9 aa, synthetic construct
GGNGNDSLE

SEQ ID NO: 25890 - protein, 9 aa, synthetic construct
GGNGNDSIY

SEQ ID NO: 25891 - protein, 9 aa, synthetic construct
GGDGADTVR

SEQ ID NO: 25892 - protein, 9 aa, synthetic construct
GGNGNDSAS

SEQ ID NO: 25893 - protein, 9 aa, synthetic construct
GGNGNDRYM

SEQ ID NO: 25894 - protein, 9 aa, synthetic construct
GGEGDDVVN

SEQ ID NO: 25895 - protein, 9 aa, synthetic construct
GGDGADVIA

SEQ ID NO: 25896 - protein, 9 aa, synthetic construct
GGGGEDTAS

SEQ ID NO: 25897 - protein, 9 aa, synthetic construct
GGNGNDRMD

SEQ ID NO: 25898 - protein, 9 aa, synthetic construct
GGNGNDRLW

SEQ ID NO: 25899 - protein, 9 aa, synthetic construct
GGDGADVFA

SEQ ID NO: 25900 - protein, 9 aa, synthetic construct
GGNGNDRIW

SEQ ID NO: 25901 - protein, 9 aa, synthetic construct
GGGGEDTFY

SEQ ID NO: 25902 - protein, 9 aa, synthetic construct
GGNGNDRAS

SEQ ID NO: 25903 - protein, 9 aa, synthetic construct
GGGGEDTIE

SEQ ID NO: 25904 - protein, 9 aa, synthetic construct
GGNGNDQYY

SEQ ID NO: 25905 - protein, 9 aa, synthetic construct
GGNGNDQVS

SEQ ID NO: 25906 - protein, 9 aa, synthetic construct
GGNGNDQVA

SEQ ID NO: 25907 - protein, 9 aa, synthetic construct
GGGGEDTLA

SEQ ID NO: 25908 - protein, 9 aa, synthetic construct
GGNGNDKLW

SEQ ID NO: 25909 - protein, 9 aa, synthetic construct
GGNGNDKLV

SEQ ID NO: 25910 - protein, 9 aa, synthetic construct
GGDGADYME

SEQ ID NO: 25911 - protein, 9 aa, synthetic construct
GGNGNDGLL

SEQ ID NO: 25912 - protein, 9 aa, synthetic construct
GGNGNDGLD

SEQ ID NO: 25913 - protein, 9 aa, synthetic construct
GGNGNDGIR

SEQ ID NO: 25914 - protein, 9 aa, synthetic construct
GGNGNDFLS

SEQ ID NO: 25915 - protein, 9 aa, synthetic construct
GGNGNDFLN

SEQ ID NO: 25916 - protein, 9 aa, synthetic construct
GGDGADYLF

SEQ ID NO: 25917 - protein, 9 aa, synthetic construct
GGNGNDFIF

SEQ ID NO: 25918 - protein, 9 aa, synthetic construct
GGDGADYLN

SEQ ID NO: 25919 - protein, 9 aa, synthetic construct
GGDGADYLQ

SEQ ID NO: 25920 - protein, 9 aa, synthetic construct
GGNGNDELR

SEQ ID NO: 25921 - protein, 9 aa, synthetic construct
GGDGADYLT

SEQ ID NO: 25922 - protein, 9 aa, synthetic construct
GGGGEDYIR

SEQ ID NO: 25923 - protein, 9 aa, synthetic construct
GGNGNDGLR

SEQ ID NO: 25924 - protein, 9 aa, synthetic construct
GGGGEDYLD

SEQ ID NO: 25925 - protein, 9 aa, synthetic construct
GGGGEDYLL

SEQ ID NO: 25926 - protein, 9 aa, synthetic construct
GGNGNDDLW

SEQ ID NO: 25927 - protein, 9 aa, synthetic construct
GGNGNDDLS

SEQ ID NO: 25928 - protein, 9 aa, synthetic construct
GGGGEDYLV

SEQ ID NO: 25929 - protein, 9 aa, synthetic construct
GGEGDDVLM

SEQ ID NO: 25930 - protein, 9 aa, synthetic construct
GGNGNDDLL

SEQ ID NO: 25931 - protein, 9 aa, synthetic construct
GGGGFDAIH

SEQ ID NO: 25932 - protein, 9 aa, synthetic construct
GGNGNDDIN

SEQ ID NO: 25933 - protein, 9 aa, synthetic construct
GGGGFDDFY

SEQ ID NO: 25934 - protein, 9 aa, synthetic construct
GGNGNDDID

SEQ ID NO: 25935 - protein, 9 aa, synthetic construct
GGNGNDGLN

SEQ ID NO: 25936 - protein, 9 aa, synthetic construct
GGDGADYIL

SEQ ID NO: 25937 - protein, 9 aa, synthetic construct
GGEGDDVVD

SEQ ID NO: 25938 - protein, 9 aa, synthetic construct
GGNGNDIVA

SEQ ID NO: 25939 - protein, 9 aa, synthetic construct
GGNGNDKLQ

SEQ ID NO: 25940 - protein, 9 aa, synthetic construct
GGNGNDKLL

SEQ ID NO: 25941 - protein, 9 aa, synthetic construct
GGGGEDTLF

SEQ ID NO: 25942 - protein, 9 aa, synthetic construct
GGDGADVVI

SEQ ID NO: 25943 - protein, 9 aa, synthetic construct
GGGGEDTLL

SEQ ID NO: 25944 - protein, 9 aa, synthetic construct
GGNGNDKID

SEQ ID NO: 25945 - protein, 9 aa, synthetic construct
GGDGADVVY

SEQ ID NO: 25946 - protein, 9 aa, synthetic construct
GGNGNDIYI

SEQ ID NO: 25947 - protein, 9 aa, synthetic construct
GGNGNDIVS

SEQ ID NO: 25948 - protein, 9 aa, synthetic construct
GGDGADWIE

SEQ ID NO: 25949 - protein, 9 aa, synthetic construct
GGDGADWIV

SEQ ID NO: 25950 - protein, 9 aa, synthetic construct
GGNGNDIMS

SEQ ID NO: 25951 - protein, 9 aa, synthetic construct
GGDGADYID

SEQ ID NO: 25952 - protein, 9 aa, synthetic construct
GGDGADWLF

SEQ ID NO: 25953 - protein, 9 aa, synthetic construct
GGNGNDILH

SEQ ID NO: 25954 - protein, 9 aa, synthetic construct
GGDGADWLG

SEQ ID NO: 25955 - protein, 9 aa, synthetic construct
GGNGNDIIN

SEQ ID NO: 25956 - protein, 9 aa, synthetic construct
GGDGADWLS

SEQ ID NO: 25957 - protein, 9 aa, synthetic construct
GGNGNDIFK

SEQ ID NO: 25958 - protein, 9 aa, synthetic construct
GGEGDDVMF

SEQ ID NO: 25959 - protein, 9 aa, synthetic construct
GGDGADWVL

SEQ ID NO: 25960 - protein, 9 aa, synthetic construct
GGNGNDHIY

SEQ ID NO: 25961 - protein, 9 aa, synthetic construct
GGDGADYFY

SEQ ID NO: 25962 - protein, 9 aa, synthetic construct
GGNGNDHIM

SEQ ID NO: 25963 - protein, 9 aa, synthetic construct
GGNGNDSYV

SEQ ID NO: 25964 - protein, 9 aa, synthetic construct
GGNGNDTAD

SEQ ID NO: 25965 - protein, 9 aa, synthetic construct
GGDGADTMA

SEQ ID NO: 25966 - protein, 9 aa, synthetic construct
GGDGADSIF

SEQ ID NO: 25967 - protein, 9 aa, synthetic construct
GGNGRDALY

SEQ ID NO: 25968 - protein, 9 aa, synthetic construct
GGDGADRVI

SEQ ID NO: 25969 - protein, 9 aa, synthetic construct
GGDGADRYI

SEQ ID NO: 25970 - protein, 9 aa, synthetic construct
GGGGEDQLA

SEQ ID NO: 25971 - protein, 9 aa, synthetic construct
GGDGADSFD

SEQ ID NO: 25972 - protein, 9 aa, synthetic construct
GGNGQDVLH

SEQ ID NO: 25973 - protein, 9 aa, synthetic construct
GGEGDDWIV

SEQ ID NO: 25974 - protein, 9 aa, synthetic construct
GGNGQDTLV

SEQ ID NO: 25975 - protein, 9 aa, synthetic construct
GGNGQDTLT

SEQ ID NO: 25976 - protein, 9 aa, synthetic construct
GGNGQDTLA

SEQ ID NO: 25977 - protein, 9 aa, synthetic construct
GGNGQDTIQ

SEQ ID NO: 25978 - protein, 9 aa, synthetic construct
GGGGEDQYL

SEQ ID NO: 25979 - protein, 9 aa, synthetic construct
GGGGEDMLY

SEQ ID NO: 25980 - protein, 9 aa, synthetic construct
GGNGQDSLD

SEQ ID NO: 25981 - protein, 9 aa, synthetic construct
GGDGADSIH

SEQ ID NO: 25982 - protein, 9 aa, synthetic construct
GGDGADSIN

SEQ ID NO: 25983 - protein, 9 aa, synthetic construct
GGNGQDLLT

SEQ ID NO: 25984 - protein, 9 aa, synthetic construct
GGNGQDLLR

SEQ ID NO: 25985 - protein, 9 aa, synthetic construct
GGNGQDKLF

SEQ ID NO: 25986 - protein, 9 aa, synthetic construct
GGNGQDIYI

SEQ ID NO: 25987 - protein, 9 aa, synthetic construct
GGNGQDHID

SEQ ID NO: 25988 - protein, 9 aa, synthetic construct
GGDGADSLK

SEQ ID NO: 25989 - protein, 9 aa, synthetic construct
GGGGEDRIR

SEQ ID NO: 25990 - protein, 9 aa, synthetic construct
GGDGADSLQ

SEQ ID NO: 25991 - protein, 9 aa, synthetic construct
GGNGRDELF

SEQ ID NO: 25992 - protein, 9 aa, synthetic construct
GGDGADRMR

SEQ ID NO: 25993 - protein, 9 aa, synthetic construct
GGDGADSLW

SEQ ID NO: 25994 - protein, 9 aa, synthetic construct
GGNGRDLLM

SEQ ID NO: 25995 - protein, 9 aa, synthetic construct
GGNGRDSIN

SEQ ID NO: 25996 - protein, 9 aa, synthetic construct
GGDGADQYF

SEQ ID NO: 25997 - protein, 9 aa, synthetic construct
GGNGRDQVY

SEQ ID NO: 25998 - protein, 9 aa, synthetic construct
GGNGRDQLY

SEQ ID NO: 25999 - protein, 9 aa, synthetic construct
GGNGRDQLR

SEQ ID NO: 26000 - protein, 9 aa, synthetic construct
GGNGRDQIS

SEQ ID NO: 26001 - protein, 9 aa, synthetic construct
GGDGADRIN

SEQ ID NO: 26002 - protein, 9 aa, synthetic construct
GGNGRDLVF

SEQ ID NO: 26003 - protein, 9 aa, synthetic construct
GGDGADRIQ

SEQ ID NO: 26004 - protein, 9 aa, synthetic construct
GGNGRDLMF

SEQ ID NO: 26005 - protein, 9 aa, synthetic construct
GGNGRDLLY

SEQ ID NO: 26006 - protein, 9 aa, synthetic construct
GGDGADRIY

SEQ ID NO: 26007 - protein, 9 aa, synthetic construct
GGNGRDFLL

SEQ ID NO: 26008 - protein, 9 aa, synthetic construct
GGNGRDLIF

SEQ ID NO: 26009 - protein, 9 aa, synthetic construct
GGNGRDLAF

SEQ ID NO: 26010 - protein, 9 aa, synthetic construct
GGNGRDKLK

SEQ ID NO: 26011 - protein, 9 aa, synthetic construct
GGGGEDKLY

SEQ ID NO: 26012 - protein, 9 aa, synthetic construct
GGNGRDKIA

SEQ ID NO: 26013 - protein, 9 aa, synthetic construct
GGNGRDKAY

SEQ ID NO: 26014 - protein, 9 aa, synthetic construct
GGNGRDIML

SEQ ID NO: 26015 - protein, 9 aa, synthetic construct
GGNGRDIMA

SEQ ID NO: 26016 - protein, 9 aa, synthetic construct
GGNGRDIAR

SEQ ID NO: 26017 - protein, 9 aa, synthetic construct
GGDGADRLW

SEQ ID NO: 26018 - protein, 9 aa, synthetic construct
GGDGADRMA

SEQ ID NO: 26019 - protein, 9 aa, synthetic construct
GGDGADSLR

SEQ ID NO: 26020 - protein, 9 aa, synthetic construct
GGDGADSVF

SEQ ID NO: 26021 - protein, 9 aa, synthetic construct
GGNGNDTAV

SEQ ID NO: 26022 - protein, 9 aa, synthetic construct
GGNGNDVIL

SEQ ID NO: 26023 - protein, 9 aa, synthetic construct
GGNGNDWFM

SEQ ID NO: 26024 - protein, 9 aa, synthetic construct
GGDGADTIG

SEQ ID NO: 26025 - protein, 9 aa, synthetic construct
GGGGEDRLV

SEQ ID NO: 26026 - protein, 9 aa, synthetic construct
GGNGNDVVF

SEQ ID NO: 26027 - protein, 9 aa, synthetic construct
GGNGNDVVD

SEQ ID NO: 26028 - protein, 9 aa, synthetic construct
GGNGNDVMA

SEQ ID NO: 26029 - protein, 9 aa, synthetic construct
GGNGNDVLQ

SEQ ID NO: 26030 - protein, 9 aa, synthetic construct
GGNGNDVLM

SEQ ID NO: 26031 - protein, 9 aa, synthetic construct
GGNGNDVIY

SEQ ID NO: 26032 - protein, 9 aa, synthetic construct
GGNGNDVIV

SEQ ID NO: 26033 - protein, 9 aa, synthetic construct
GGNGNDVIR

SEQ ID NO: 26034 - protein, 9 aa, synthetic construct
GGNGNDVIF

SEQ ID NO: 26035 - protein, 9 aa, synthetic construct
GGNGNDWLI

SEQ ID NO: 26036 - protein, 9 aa, synthetic construct
GGNGNDVFQ

SEQ ID NO: 26037 - protein, 9 aa, synthetic construct
GGDGADTIW

SEQ ID NO: 26038 - protein, 9 aa, synthetic construct
GGNGNDTYQ

SEQ ID NO: 26039 - protein, 9 aa, synthetic construct
GGNGNDTYH

SEQ ID NO: 26040 - protein, 9 aa, synthetic construct
GGNGNDTYG

SEQ ID NO: 26041 - protein, 9 aa, synthetic construct
GGNGNDTVM

SEQ ID NO: 26042 - protein, 9 aa, synthetic construct
GGNGNDTVG

SEQ ID NO: 26043 - protein, 9 aa, synthetic construct
GGNGNDTVA

SEQ ID NO: 26044 - protein, 9 aa, synthetic construct
GGNGNDTME

SEQ ID NO: 26045 - protein, 9 aa, synthetic construct
GGNGNDTIG

SEQ ID NO: 26046 - protein, 9 aa, synthetic construct
GGNGNDTFF

SEQ ID NO: 26047 - protein, 9 aa, synthetic construct
GGNGNDWLF

SEQ ID NO: 26048 - protein, 9 aa, synthetic construct
GGNGNDWLL

SEQ ID NO: 26049 - protein, 9 aa, synthetic construct
GGDGADSVH

SEQ ID NO: 26050 - protein, 9 aa, synthetic construct
GGDGADSYM

SEQ ID NO: 26051 - protein, 9 aa, synthetic construct
GGDGADSVI

SEQ ID NO: 26052 - protein, 9 aa, synthetic construct
GGDGADSVL

SEQ ID NO: 26053 - protein, 9 aa, synthetic construct
GGDGADSVR

SEQ ID NO: 26054 - protein, 9 aa, synthetic construct
GGNGPDILV

SEQ ID NO: 26055 - protein, 9 aa, synthetic construct
GGNGPDILK

SEQ ID NO: 26056 - protein, 9 aa, synthetic construct
GGEGDDWAA

SEQ ID NO: 26057 - protein, 9 aa, synthetic construct
GGNGNDYVT

SEQ ID NO: 26058 - protein, 9 aa, synthetic construct
GGNGNDYMS

SEQ ID NO: 26059 - protein, 9 aa, synthetic construct
GGNGNDYML

SEQ ID NO: 26060 - protein, 9 aa, synthetic construct
GGDGADSVW

SEQ ID NO: 26061 - protein, 9 aa, synthetic construct
GGDGADSYA

SEQ ID NO: 26062 - protein, 9 aa, synthetic construct
GGNGNDYLS

SEQ ID NO: 26063 - protein, 9 aa, synthetic construct
GGNGNDWLV

SEQ ID NO: 26064 - protein, 9 aa, synthetic construct
GGNGNDYLL

SEQ ID NO: 26065 - protein, 9 aa, synthetic construct
GGDGADTAS

SEQ ID NO: 26066 - protein, 9 aa, synthetic construct
GGNGNDYLA

SEQ ID NO: 26067 - protein, 9 aa, synthetic construct
GGNGNDYIY

SEQ ID NO: 26068 - protein, 9 aa, synthetic construct
GGGGEDRLE

SEQ ID NO: 26069 - protein, 9 aa, synthetic construct
GGGGEDRLL

SEQ ID NO: 26070 - protein, 9 aa, synthetic construct
GGNGNDYID

SEQ ID NO: 26071 - protein, 9 aa, synthetic construct
GGDGADTFG

SEQ ID NO: 26072 - protein, 9 aa, synthetic construct
GGNGNDYAL

SEQ ID NO: 26073 - protein, 9 aa, synthetic construct
GGNGNDYAD

SEQ ID NO: 26074 - protein, 9 aa, synthetic construct
GGNGNDWLY

SEQ ID NO: 26075 - protein, 9 aa, synthetic construct
GGNGNDDIA

SEQ ID NO: 26076 - protein, 9 aa, synthetic construct
GGGGFDEMY

SEQ ID NO: 26077 - protein, 9 aa, synthetic construct
GGNGEDDLT

SEQ ID NO: 26078 - protein, 9 aa, synthetic construct
GGEGDDVLG

SEQ ID NO: 26079 - protein, 9 aa, synthetic construct
GGNGGDVLD

SEQ ID NO: 26080 - protein, 9 aa, synthetic construct
GGDGDDGLY

SEQ ID NO: 26081 - protein, 9 aa, synthetic construct
GGNGGDTYV

SEQ ID NO: 26082 - protein, 9 aa, synthetic construct
GGGGGDAMA

SEQ ID NO: 26083 - protein, 9 aa, synthetic construct
GGGGGDAVD

SEQ ID NO: 26084 - protein, 9 aa, synthetic construct
GGNGGDTLS

SEQ ID NO: 26085 - protein, 9 aa, synthetic construct
GGNGGDTLL

SEQ ID NO: 26086 - protein, 9 aa, synthetic construct
GGEGDDTVY

SEQ ID NO: 26087 - protein, 9 aa, synthetic construct
GGDGDDHIH

SEQ ID NO: 26088 - protein, 9 aa, synthetic construct
GGNGGDTIY

SEQ ID NO: 26089 - protein, 9 aa, synthetic construct
GGDGDDHIL

SEQ ID NO: 26090 - protein, 9 aa, synthetic construct
GGGGGDDIN

SEQ ID NO: 26091 - protein, 9 aa, synthetic construct
GGDGDDHIV

SEQ ID NO: 26092 - protein, 9 aa, synthetic construct
GGNGGDSLA

SEQ ID NO: 26093 - protein, 9 aa, synthetic construct
GGNGGDSIL

SEQ ID NO: 26094 - protein, 9 aa, synthetic construct
GGDGDDHIY

SEQ ID NO: 26095 - protein, 9 aa, synthetic construct
GGGGGDDLF

SEQ ID NO: 26096 - protein, 9 aa, synthetic construct
GGGGGDDLG

SEQ ID NO: 26097 - protein, 9 aa, synthetic construct
GGEGDDTVT

SEQ ID NO: 26098 - protein, 9 aa, synthetic construct
GGNGGDNLT

SEQ ID NO: 26099 - protein, 9 aa, synthetic construct
GGDGDDHML

SEQ ID NO: 26100 - protein, 9 aa, synthetic construct
GGNGGDLLT

SEQ ID NO: 26101 - protein, 9 aa, synthetic construct
GGNGGDLLS

SEQ ID NO: 26102 - protein, 9 aa, synthetic construct
GGNGGDLLI

SEQ ID NO: 26103 - protein, 9 aa, synthetic construct
GGNGGDLLH

SEQ ID NO: 26104 - protein, 9 aa, synthetic construct
GGGGGDALY

SEQ ID NO: 26105 - protein, 9 aa, synthetic construct
GGDGDDGLT

SEQ ID NO: 26106 - protein, 9 aa, synthetic construct
GGDGDDGLR

SEQ ID NO: 26107 - protein, 9 aa, synthetic construct
GGDGDDFVT

SEQ ID NO: 26108 - protein, 9 aa, synthetic construct
GGDGDDFMG

SEQ ID NO: 26109 - protein, 9 aa, synthetic construct
GGNGHDLLL

SEQ ID NO: 26110 - protein, 9 aa, synthetic construct
GGDGDDFVA

SEQ ID NO: 26111 - protein, 9 aa, synthetic construct
GGNGHDLIL

SEQ ID NO: 26112 - protein, 9 aa, synthetic construct
GGNGHDLFS

SEQ ID NO: 26113 - protein, 9 aa, synthetic construct
GGDGDDFVE

SEQ ID NO: 26114 - protein, 9 aa, synthetic construct
GGNGHDKLF

SEQ ID NO: 26115 - protein, 9 aa, synthetic construct
GGNGHDIYY

SEQ ID NO: 26116 - protein, 9 aa, synthetic construct
GGGGFDTYY

SEQ ID NO: 26117 - protein, 9 aa, synthetic construct
GGNGHDIIL

SEQ ID NO: 26118 - protein, 9 aa, synthetic construct
GGDGDDFVR

SEQ ID NO: 26119 - protein, 9 aa, synthetic construct
GGNGHDHLN

SEQ ID NO: 26120 - protein, 9 aa, synthetic construct
GGGGGDALG

SEQ ID NO: 26121 - protein, 9 aa, synthetic construct
GGDGDDFVV

SEQ ID NO: 26122 - protein, 9 aa, synthetic construct
GGDGDDFYV

SEQ ID NO: 26123 - protein, 9 aa, synthetic construct
GGDGDDGIN

SEQ ID NO: 26124 - protein, 9 aa, synthetic construct
GGEGDDTYR

SEQ ID NO: 26125 - protein, 9 aa, synthetic construct
GGNGHDDLQ

SEQ ID NO: 26126 - protein, 9 aa, synthetic construct
GGEGDDTYL

SEQ ID NO: 26127 - protein, 9 aa, synthetic construct
GGDGDDGLA

SEQ ID NO: 26128 - protein, 9 aa, synthetic construct
GGEGDDTYF

SEQ ID NO: 26129 - protein, 9 aa, synthetic construct
GGDGDDGLL

SEQ ID NO: 26130 - protein, 9 aa, synthetic construct
GGNGGDVVI

SEQ ID NO: 26131 - protein, 9 aa, synthetic construct
GGNGGDVVD

SEQ ID NO: 26132 - protein, 9 aa, synthetic construct
GGEGDDTVF

SEQ ID NO: 26133 - protein, 9 aa, synthetic construct
GGEGDDTVE

SEQ ID NO: 26134 - protein, 9 aa, synthetic construct
GGDGDDIAY

SEQ ID NO: 26135 - protein, 9 aa, synthetic construct
GGNGEDRFV

SEQ ID NO: 26136 - protein, 9 aa, synthetic construct
GGNGEDTLV

SEQ ID NO: 26137 - protein, 9 aa, synthetic construct
GGNGEDTLT

SEQ ID NO: 26138 - protein, 9 aa, synthetic construct
GGNGEDTLQ

SEQ ID NO: 26139 - protein, 9 aa, synthetic construct
GGNGEDTLL

SEQ ID NO: 26140 - protein, 9 aa, synthetic construct
GGDGDDIYF

SEQ ID NO: 26141 - protein, 9 aa, synthetic construct
GGGGGDILL

SEQ ID NO: 26142 - protein, 9 aa, synthetic construct
GGNGEDSVN

SEQ ID NO: 26143 - protein, 9 aa, synthetic construct
GGNGEDSLV

SEQ ID NO: 26144 - protein, 9 aa, synthetic construct
GGNGEDRLV

SEQ ID NO: 26145 - protein, 9 aa, synthetic construct
GGDGDDKAY

SEQ ID NO: 26146 - protein, 9 aa, synthetic construct
GGNGEDRID

SEQ ID NO: 26147 - protein, 9 aa, synthetic construct
GGDGDDKIF

SEQ ID NO: 26148 - protein, 9 aa, synthetic construct
GGDGDDIVI

SEQ ID NO: 26149 - protein, 9 aa, synthetic construct
GGDGDDKIH

SEQ ID NO: 26150 - protein, 9 aa, synthetic construct
GGNGEDNIL

SEQ ID NO: 26151 - protein, 9 aa, synthetic construct
GGNGEDLLA

SEQ ID NO: 26152 - protein, 9 aa, synthetic construct
GGDGDDKIT

SEQ ID NO: 26153 - protein, 9 aa, synthetic construct
GGDGDDKIV

SEQ ID NO: 26154 - protein, 9 aa, synthetic construct
GGDGDDKIY

SEQ ID NO: 26155 - protein, 9 aa, synthetic construct
GGNGEDILD

SEQ ID NO: 26156 - protein, 9 aa, synthetic construct
GGGGGDIVV

SEQ ID NO: 26157 - protein, 9 aa, synthetic construct
GGNGEDHVF

SEQ ID NO: 26158 - protein, 9 aa, synthetic construct
GGDGDDKLK

SEQ ID NO: 26159 - protein, 9 aa, synthetic construct
GGDGDDKLL

SEQ ID NO: 26160 - protein, 9 aa, synthetic construct
GGDGDDIVL

SEQ ID NO: 26161 - protein, 9 aa, synthetic construct
GGNGEDYID

SEQ ID NO: 26162 - protein, 9 aa, synthetic construct
GGDGDDIFG

SEQ ID NO: 26163 - protein, 9 aa, synthetic construct
GGNGFDTVD

SEQ ID NO: 26164 - protein, 9 aa, synthetic construct
GGNGGDHVD

SEQ ID NO: 26165 - protein, 9 aa, synthetic construct
GGDGDDIFY

SEQ ID NO: 26166 - protein, 9 aa, synthetic construct
GGNGGDDYM

SEQ ID NO: 26167 - protein, 9 aa, synthetic construct
GGNGGDDLS

SEQ ID NO: 26168 - protein, 9 aa, synthetic construct
GGNGGDDLM

SEQ ID NO: 26169 - protein, 9 aa, synthetic construct
GGNGGDALD

SEQ ID NO: 26170 - protein, 9 aa, synthetic construct
GGNGGDAIY

SEQ ID NO: 26171 - protein, 9 aa, synthetic construct
GGNGFDVLD

SEQ ID NO: 26172 - protein, 9 aa, synthetic construct
GGDGDDIIK

SEQ ID NO: 26173 - protein, 9 aa, synthetic construct
GGNGFDTYL

SEQ ID NO: 26174 - protein, 9 aa, synthetic construct
GGDGDDIIL

SEQ ID NO: 26175 - protein, 9 aa, synthetic construct
GGNGFDSLV

SEQ ID NO: 26176 - protein, 9 aa, synthetic construct
GGGGGDHLV

SEQ ID NO: 26177 - protein, 9 aa, synthetic construct
GGNGFDRID

SEQ ID NO: 26178 - protein, 9 aa, synthetic construct
GGNGFDRAR

SEQ ID NO: 26179 - protein, 9 aa, synthetic construct
GGNGFDLLD

SEQ ID NO: 26180 - protein, 9 aa, synthetic construct
GGNGFDKFI

SEQ ID NO: 26181 - protein, 9 aa, synthetic construct
GGNGFDIAS

SEQ ID NO: 26182 - protein, 9 aa, synthetic construct
GGNGFDIAM

SEQ ID NO: 26183 - protein, 9 aa, synthetic construct
GGEGDDTMT

SEQ ID NO: 26184 - protein, 9 aa, synthetic construct
GGDGDDIMG

SEQ ID NO: 26185 - protein, 9 aa, synthetic construct
GGEGDDTMG

SEQ ID NO: 26186 - protein, 9 aa, synthetic construct
GGGGGDHLI

SEQ ID NO: 26187 - protein, 9 aa, synthetic construct
GGGGGDHLS

SEQ ID NO: 26188 - protein, 9 aa, synthetic construct
GGNGHDLLY

SEQ ID NO: 26189 - protein, 9 aa, synthetic construct
GGNGHDMLF

SEQ ID NO: 26190 - protein, 9 aa, synthetic construct
GGNGHDMLQ

SEQ ID NO: 26191 - protein, 9 aa, synthetic construct
GGDGDDDIL

SEQ ID NO: 26192 - protein, 9 aa, synthetic construct
GGDGDDCLT

SEQ ID NO: 26193 - protein, 9 aa, synthetic construct
GGNGKDYLD

SEQ ID NO: 26194 - protein, 9 aa, synthetic construct
GGDGDDDFR

SEQ ID NO: 26195 - protein, 9 aa, synthetic construct
GGNGKDVLN

SEQ ID NO: 26196 - protein, 9 aa, synthetic construct
GGNGKDVFV

SEQ ID NO: 26197 - protein, 9 aa, synthetic construct
GGGGFDRAV

SEQ ID NO: 26198 - protein, 9 aa, synthetic construct
GGNGKDTVI

SEQ ID NO: 26199 - protein, 9 aa, synthetic construct
GGNGKDTLV

SEQ ID NO: 26200 - protein, 9 aa, synthetic construct
GGNGKDTLT

SEQ ID NO: 26201 - protein, 9 aa, synthetic construct
GGNGKDTLK

SEQ ID NO: 26202 - protein, 9 aa, synthetic construct
GGNGKDTLI

SEQ ID NO: 26203 - protein, 9 aa, synthetic construct
GGDGDDDIN

SEQ ID NO: 26204 - protein, 9 aa, synthetic construct
GGNGLDILY

SEQ ID NO: 26205 - protein, 9 aa, synthetic construct
GGNGKDTLD

SEQ ID NO: 26206 - protein, 9 aa, synthetic construct
GGNGKDTIY

SEQ ID NO: 26207 - protein, 9 aa, synthetic construct
GGNGKDTIN

SEQ ID NO: 26208 - protein, 9 aa, synthetic construct
GGNGKDTIF

SEQ ID NO: 26209 - protein, 9 aa, synthetic construct
GGGGFDRLD

SEQ ID NO: 26210 - protein, 9 aa, synthetic construct
GGDGDDDIY

SEQ ID NO: 26211 - protein, 9 aa, synthetic construct
GGDGDDDLI

SEQ ID NO: 26212 - protein, 9 aa, synthetic construct
GGNGKDRID

SEQ ID NO: 26213 - protein, 9 aa, synthetic construct
GGNGKDNLQ

SEQ ID NO: 26214 - protein, 9 aa, synthetic construct
GGNGKDLLQ

SEQ ID NO: 26215 - protein, 9 aa, synthetic construct
GGNGKDLLN

SEQ ID NO: 26216 - protein, 9 aa, synthetic construct
GGDGDDCIE

SEQ ID NO: 26217 - protein, 9 aa, synthetic construct
GGNGLDKLY

SEQ ID NO: 26218 - protein, 9 aa, synthetic construct
GGNGKDLLD

SEQ ID NO: 26219 - protein, 9 aa, synthetic construct
GGNGLDVIS

SEQ ID NO: 26220 - protein, 9 aa, synthetic construct
GGNGNDAMY

SEQ ID NO: 26221 - protein, 9 aa, synthetic construct
GGNGNDAMR

SEQ ID NO: 26222 - protein, 9 aa, synthetic construct
GGNGNDAIN

SEQ ID NO: 26223 - protein, 9 aa, synthetic construct
GGNGMDTYE

SEQ ID NO: 26224 - protein, 9 aa, synthetic construct
GGDGDDAIL

SEQ ID NO: 26225 - protein, 9 aa, synthetic construct
GGGGFDIMN

SEQ ID NO: 26226 - protein, 9 aa, synthetic construct
GGNGMDSFV

SEQ ID NO: 26227 - protein, 9 aa, synthetic construct
GGNGMDQLY

SEQ ID NO: 26228 - protein, 9 aa, synthetic construct
GGDGDDAIW

SEQ ID NO: 26229 - protein, 9 aa, synthetic construct
GGNGMDLLD

SEQ ID NO: 26230 - protein, 9 aa, synthetic construct
GGNGLDYYY

SEQ ID NO: 26231 - protein, 9 aa, synthetic construct
GGNGLDTLR

SEQ ID NO: 26232 - protein, 9 aa, synthetic construct
GGGGFDLLV

SEQ ID NO: 26233 - protein, 9 aa, synthetic construct
GGNGLDTLN

SEQ ID NO: 26234 - protein, 9 aa, synthetic construct
GGNGLDTIL

SEQ ID NO: 26235 - protein, 9 aa, synthetic construct
GGNGLDSLD

SEQ ID NO: 26236 - protein, 9 aa, synthetic construct
GGDGDDAMG

SEQ ID NO: 26237 - protein, 9 aa, synthetic construct
GGDGDDAMH

SEQ ID NO: 26238 - protein, 9 aa, synthetic construct
GGDGDDAMS

SEQ ID NO: 26239 - protein, 9 aa, synthetic construct
GGNGLDQLS

SEQ ID NO: 26240 - protein, 9 aa, synthetic construct
GGDGDDAMY

SEQ ID NO: 26241 - protein, 9 aa, synthetic construct
GGNGLDLLY

SEQ ID NO: 26242 - protein, 9 aa, synthetic construct
GGDGDDAVF

SEQ ID NO: 26243 - protein, 9 aa, synthetic construct
GGNGLDLLQ

SEQ ID NO: 26244 - protein, 9 aa, synthetic construct
GGNGKDLLI

SEQ ID NO: 26245 - protein, 9 aa, synthetic construct
GGNGKDKVI

SEQ ID NO: 26246 - protein, 9 aa, synthetic construct
GGNGHDRLF

SEQ ID NO: 26247 - protein, 9 aa, synthetic construct
GGDGDDFIE

SEQ ID NO: 26248 - protein, 9 aa, synthetic construct
GGDGDDELT

SEQ ID NO: 26249 - protein, 9 aa, synthetic construct
GGEGDDVFV

SEQ ID NO: 26250 - protein, 9 aa, synthetic construct
GGNGIDFLT

SEQ ID NO: 26251 - protein, 9 aa, synthetic construct
GGNGIDFLI

SEQ ID NO: 26252 - protein, 9 aa, synthetic construct
GGGGFDTFV

SEQ ID NO: 26253 - protein, 9 aa, synthetic construct
GGNGIDALS

SEQ ID NO: 26254 - protein, 9 aa, synthetic construct
GGDGDDEVH

SEQ ID NO: 26255 - protein, 9 aa, synthetic construct
GGGGFDTIT

SEQ ID NO: 26256 - protein, 9 aa, synthetic construct
GGNGHDYID

SEQ ID NO: 26257 - protein, 9 aa, synthetic construct
GGDGDDFAK

SEQ ID NO: 26258 - protein, 9 aa, synthetic construct
GGGGFDTLN

SEQ ID NO: 26259 - protein, 9 aa, synthetic construct
GGGGFDTLT

SEQ ID NO: 26260 - protein, 9 aa, synthetic construct
GGNGIDMAH

SEQ ID NO: 26261 - protein, 9 aa, synthetic construct
GGDGDDFIH

SEQ ID NO: 26262 - protein, 9 aa, synthetic construct
GGGGFDTLV

SEQ ID NO: 26263 - protein, 9 aa, synthetic construct
GGNGHDTLM

SEQ ID NO: 26264 - protein, 9 aa, synthetic construct
GGNGHDTLH

SEQ ID NO: 26265 - protein, 9 aa, synthetic construct
GGNGHDTLF

SEQ ID NO: 26266 - protein, 9 aa, synthetic construct
GGNGHDSLY

SEQ ID NO: 26267 - protein, 9 aa, synthetic construct
GGDGDDFIT

SEQ ID NO: 26268 - protein, 9 aa, synthetic construct
GGNGHDSIA

SEQ ID NO: 26269 - protein, 9 aa, synthetic construct
GGDGDDFLG

SEQ ID NO: 26270 - protein, 9 aa, synthetic construct
GGNGHDRLL

SEQ ID NO: 26271 - protein, 9 aa, synthetic construct
GGNGHDRLI

SEQ ID NO: 26272 - protein, 9 aa, synthetic construct
GGNGIDKLY

SEQ ID NO: 26273 - protein, 9 aa, synthetic construct
GGDGDDELM

SEQ ID NO: 26274 - protein, 9 aa, synthetic construct
GGNGKDKLA

SEQ ID NO: 26275 - protein, 9 aa, synthetic construct
GGNGIDVLD

SEQ ID NO: 26276 - protein, 9 aa, synthetic construct
GGDGDDDLV

SEQ ID NO: 26277 - protein, 9 aa, synthetic construct
GGNGKDHLT

SEQ ID NO: 26278 - protein, 9 aa, synthetic construct
GGDGDDDLW

SEQ ID NO: 26279 - protein, 9 aa, synthetic construct
GGDGDDDLY

SEQ ID NO: 26280 - protein, 9 aa, synthetic construct
GGGGFDRLT

SEQ ID NO: 26281 - protein, 9 aa, synthetic construct
GGNGKDALR

SEQ ID NO: 26282 - protein, 9 aa, synthetic construct
GGDGDDDVI

SEQ ID NO: 26283 - protein, 9 aa, synthetic construct
GGGGFDRVD

SEQ ID NO: 26284 - protein, 9 aa, synthetic construct
GGNGIDWLQ

SEQ ID NO: 26285 - protein, 9 aa, synthetic construct
GGGGFDRVS

SEQ ID NO: 26286 - protein, 9 aa, synthetic construct
GGNGIDVLS

SEQ ID NO: 26287 - protein, 9 aa, synthetic construct
GGNGIDVLA

SEQ ID NO: 26288 - protein, 9 aa, synthetic construct
GGDGDDELK

SEQ ID NO: 26289 - protein, 9 aa, synthetic construct
GGNGIDTYD

SEQ ID NO: 26290 - protein, 9 aa, synthetic construct
GGDGDDDYT

SEQ ID NO: 26291 - protein, 9 aa, synthetic construct
GGNGIDTVM

SEQ ID NO: 26292 - protein, 9 aa, synthetic construct
GGDGDDEIA

SEQ ID NO: 26293 - protein, 9 aa, synthetic construct
GGNGIDTIS

SEQ ID NO: 26294 - protein, 9 aa, synthetic construct
GGDGDDEIK

SEQ ID NO: 26295 - protein, 9 aa, synthetic construct
GGNGIDTIN

SEQ ID NO: 26296 - protein, 9 aa, synthetic construct
GGGGFDTAD

SEQ ID NO: 26297 - protein, 9 aa, synthetic construct
GGNGIDTAL

SEQ ID NO: 26298 - protein, 9 aa, synthetic construct
GGDGDDEIW

SEQ ID NO: 26299 - protein, 9 aa, synthetic construct
GGNGIDRMT

SEQ ID NO: 26300 - protein, 9 aa, synthetic construct
GGGGDDDYV

SEQ ID NO: 26301 - protein, 9 aa, synthetic construct
GGPGRDILI

SEQ ID NO: 26302 - protein, 9 aa, synthetic construct
GGQGDDAIY

SEQ ID NO: 26303 - protein, 9 aa, synthetic construct
GGEGGDWLV

SEQ ID NO: 26304 - protein, 9 aa, synthetic construct
GGRGEDTLD

SEQ ID NO: 26305 - protein, 9 aa, synthetic construct
GGRGEDTIF

SEQ ID NO: 26306 - protein, 9 aa, synthetic construct
GGRGEDTIE

SEQ ID NO: 26307 - protein, 9 aa, synthetic construct
GGRGEDTFV

SEQ ID NO: 26308 - protein, 9 aa, synthetic construct
GGRGEDRLL

SEQ ID NO: 26309 - protein, 9 aa, synthetic construct
GGRGEDRLI

SEQ ID NO: 26310 - protein, 9 aa, synthetic construct
GGEGGDWLN

SEQ ID NO: 26311 - protein, 9 aa, synthetic construct
GGRGEDLLY

SEQ ID NO: 26312 - protein, 9 aa, synthetic construct
GGAGRDKMI

SEQ ID NO: 26313 - protein, 9 aa, synthetic construct
GGRGEDILN

SEQ ID NO: 26314 - protein, 9 aa, synthetic construct
GGAGRDKMY

SEQ ID NO: 26315 - protein, 9 aa, synthetic construct
GGRGEDFLF

SEQ ID NO: 26316 - protein, 9 aa, synthetic construct
GGRGEDEMV

SEQ ID NO: 26317 - protein, 9 aa, synthetic construct
GGRGEDAVD

SEQ ID NO: 26318 - protein, 9 aa, synthetic construct
GGRGDDYYQ

SEQ ID NO: 26319 - protein, 9 aa, synthetic construct
GGEGGDVMR

SEQ ID NO: 26320 - protein, 9 aa, synthetic construct
GGRGDDYLW

SEQ ID NO: 26321 - protein, 9 aa, synthetic construct
GGAGRDLIE

SEQ ID NO: 26322 - protein, 9 aa, synthetic construct
GGRGDDYLS

SEQ ID NO: 26323 - protein, 9 aa, synthetic construct
GGRGDDYLL

SEQ ID NO: 26324 - protein, 9 aa, synthetic construct
GGGGADLMD

SEQ ID NO: 26325 - protein, 9 aa, synthetic construct
GGGGADLMH

SEQ ID NO: 26326 - protein, 9 aa, synthetic construct
GGGGADLMI

SEQ ID NO: 26327 - protein, 9 aa, synthetic construct
GGAGRDKIE

SEQ ID NO: 26328 - protein, 9 aa, synthetic construct
GGRGEDVIR

SEQ ID NO: 26329 - protein, 9 aa, synthetic construct
GGRGDDVVS

SEQ ID NO: 26330 - protein, 9 aa, synthetic construct
GGEGGDYFF

SEQ ID NO: 26331 - protein, 9 aa, synthetic construct
GGRGGDRLS

SEQ ID NO: 26332 - protein, 9 aa, synthetic construct
GGRGGDRLI

SEQ ID NO: 26333 - protein, 9 aa, synthetic construct
GGAGRDIIY

SEQ ID NO: 26334 - protein, 9 aa, synthetic construct
GGRGGDQMI

SEQ ID NO: 26335 - protein, 9 aa, synthetic construct
GGAGRDILG

SEQ ID NO: 26336 - protein, 9 aa, synthetic construct
GGRGGDLLI

SEQ ID NO: 26337 - protein, 9 aa, synthetic construct
GGAGRDILK

SEQ ID NO: 26338 - protein, 9 aa, synthetic construct
GGAGRDILQ

SEQ ID NO: 26339 - protein, 9 aa, synthetic construct
GGAGRDILR

SEQ ID NO: 26340 - protein, 9 aa, synthetic construct
GGRGGDAFV

SEQ ID NO: 26341 - protein, 9 aa, synthetic construct
GGAGRDILW

SEQ ID NO: 26342 - protein, 9 aa, synthetic construct
GGRGFDTLD

SEQ ID NO: 26343 - protein, 9 aa, synthetic construct
GGRGFDTIQ

SEQ ID NO: 26344 - protein, 9 aa, synthetic construct
GGAGRDIMI

SEQ ID NO: 26345 - protein, 9 aa, synthetic construct
GGRGFDRLT

SEQ ID NO: 26346 - protein, 9 aa, synthetic construct
GGRGFDMLQ

SEQ ID NO: 26347 - protein, 9 aa, synthetic construct
GGRGFDMLM

SEQ ID NO: 26348 - protein, 9 aa, synthetic construct
GGAGRDIVA

SEQ ID NO: 26349 - protein, 9 aa, synthetic construct
GGAGRDIVQ

SEQ ID NO: 26350 - protein, 9 aa, synthetic construct
GGAGRDIVS

SEQ ID NO: 26351 - protein, 9 aa, synthetic construct
GGRGEDYLE

SEQ ID NO: 26352 - protein, 9 aa, synthetic construct
GGRGEDVLY

SEQ ID NO: 26353 - protein, 9 aa, synthetic construct
GGRGEDVLV

SEQ ID NO: 26354 - protein, 9 aa, synthetic construct
GGAGRDLIN

SEQ ID NO: 26355 - protein, 9 aa, synthetic construct
GGRGDDVVD

SEQ ID NO: 26356 - protein, 9 aa, synthetic construct
GGEGHDILI

SEQ ID NO: 26357 - protein, 9 aa, synthetic construct
GGAGRDMIY

SEQ ID NO: 26358 - protein, 9 aa, synthetic construct
GGRGDDSLA

SEQ ID NO: 26359 - protein, 9 aa, synthetic construct
GGGGADLYG

SEQ ID NO: 26360 - protein, 9 aa, synthetic construct
GGEGGDVFQ

SEQ ID NO: 26361 - protein, 9 aa, synthetic construct
GGRGDDRYV

SEQ ID NO: 26362 - protein, 9 aa, synthetic construct
GGRGDDRMT

SEQ ID NO: 26363 - protein, 9 aa, synthetic construct
GGGGADMFR

SEQ ID NO: 26364 - protein, 9 aa, synthetic construct
GGRGDDRLN

SEQ ID NO: 26365 - protein, 9 aa, synthetic construct
GGRGDDRLK

SEQ ID NO: 26366 - protein, 9 aa, synthetic construct
GGEGGDVFA

SEQ ID NO: 26367 - protein, 9 aa, synthetic construct
GGRGDDRIS

SEQ ID NO: 26368 - protein, 9 aa, synthetic construct
GGAGRDNIW

SEQ ID NO: 26369 - protein, 9 aa, synthetic construct
GGAGRDNLE

SEQ ID NO: 26370 - protein, 9 aa, synthetic construct
GGGGADMLD

SEQ ID NO: 26371 - protein, 9 aa, synthetic construct
GGAGRDNLV

SEQ ID NO: 26372 - protein, 9 aa, synthetic construct
GGGGADMLG

SEQ ID NO: 26373 - protein, 9 aa, synthetic construct
GGRGDDQLV

SEQ ID NO: 26374 - protein, 9 aa, synthetic construct
GGRGDDQLT

SEQ ID NO: 26375 - protein, 9 aa, synthetic construct
GGRGDDQLI

SEQ ID NO: 26376 - protein, 9 aa, synthetic construct
GGRGDDQLF

SEQ ID NO: 26377 - protein, 9 aa, synthetic construct
GGRGDDQLE

SEQ ID NO: 26378 - protein, 9 aa, synthetic construct
GGEGGDTVC

SEQ ID NO: 26379 - protein, 9 aa, synthetic construct
GGAGRDQFL

SEQ ID NO: 26380 - protein, 9 aa, synthetic construct
GGGGADMLM

SEQ ID NO: 26381 - protein, 9 aa, synthetic construct
GGAGRDMLA

SEQ ID NO: 26382 - protein, 9 aa, synthetic construct
GGRGDDSLM

SEQ ID NO: 26383 - protein, 9 aa, synthetic construct
GGAGRDLLH

SEQ ID NO: 26384 - protein, 9 aa, synthetic construct
GGRGDDSLR

SEQ ID NO: 26385 - protein, 9 aa, synthetic construct
GGRGDDVLQ

SEQ ID NO: 26386 - protein, 9 aa, synthetic construct
GGRGDDVLK

SEQ ID NO: 26387 - protein, 9 aa, synthetic construct
GGRGDDVLH

SEQ ID NO: 26388 - protein, 9 aa, synthetic construct
GGRGDDVIY

SEQ ID NO: 26389 - protein, 9 aa, synthetic construct
GGRGDDVIT

SEQ ID NO: 26390 - protein, 9 aa, synthetic construct
GGRGDDVIH

SEQ ID NO: 26391 - protein, 9 aa, synthetic construct
GGRGDDVFV

SEQ ID NO: 26392 - protein, 9 aa, synthetic construct
GGRGDDTYY

SEQ ID NO: 26393 - protein, 9 aa, synthetic construct
GGRGDDTVL

SEQ ID NO: 26394 - protein, 9 aa, synthetic construct
GGGGADLMV

SEQ ID NO: 26395 - protein, 9 aa, synthetic construct
GGAGRDLMD

SEQ ID NO: 26396 - protein, 9 aa, synthetic construct
GGRGDDTVF

SEQ ID NO: 26397 - protein, 9 aa, synthetic construct
GGAGRDLMH

SEQ ID NO: 26398 - protein, 9 aa, synthetic construct
GGRGDDTMT

SEQ ID NO: 26399 - protein, 9 aa, synthetic construct
GGAGRDLMW

SEQ ID NO: 26400 - protein, 9 aa, synthetic construct
GGRGDDTIT

SEQ ID NO: 26401 - protein, 9 aa, synthetic construct
GGRGDDTIM

SEQ ID NO: 26402 - protein, 9 aa, synthetic construct
GGRGDDTII

SEQ ID NO: 26403 - protein, 9 aa, synthetic construct
GGRGDDTIG

SEQ ID NO: 26404 - protein, 9 aa, synthetic construct
GGRGDDTIE

SEQ ID NO: 26405 - protein, 9 aa, synthetic construct
GGRGDDSVS

SEQ ID NO: 26406 - protein, 9 aa, synthetic construct
GGAGRDMAV

SEQ ID NO: 26407 - protein, 9 aa, synthetic construct
GGRGDDSLV

SEQ ID NO: 26408 - protein, 9 aa, synthetic construct
GGRGGDRVA

SEQ ID NO: 26409 - protein, 9 aa, synthetic construct
GGAGRDIFY

SEQ ID NO: 26410 - protein, 9 aa, synthetic construct
GGAGRDIFV

SEQ ID NO: 26411 - protein, 9 aa, synthetic construct
GGAGRDCFV

SEQ ID NO: 26412 - protein, 9 aa, synthetic construct
GGAGRDDIN

SEQ ID NO: 26413 - protein, 9 aa, synthetic construct
GGRGKDQLQ

SEQ ID NO: 26414 - protein, 9 aa, synthetic construct
GGGGADIMI

SEQ ID NO: 26415 - protein, 9 aa, synthetic construct
GGRGKDLLS

SEQ ID NO: 26416 - protein, 9 aa, synthetic construct
GGEGHDHMD

SEQ ID NO: 26417 - protein, 9 aa, synthetic construct
GGRGKDLLF

SEQ ID NO: 26418 - protein, 9 aa, synthetic construct
GGRGKDKMN

SEQ ID NO: 26419 - protein, 9 aa, synthetic construct
GGRGKDKLN

SEQ ID NO: 26420 - protein, 9 aa, synthetic construct
GGAGRDDLY

SEQ ID NO: 26421 - protein, 9 aa, synthetic construct
GGGGADIVL

SEQ ID NO: 26422 - protein, 9 aa, synthetic construct
GGEGHDFLA

SEQ ID NO: 26423 - protein, 9 aa, synthetic construct
GGGGADKAW

SEQ ID NO: 26424 - protein, 9 aa, synthetic construct
GGRGKDELR

SEQ ID NO: 26425 - protein, 9 aa, synthetic construct
GGAGRDEID

SEQ ID NO: 26426 - protein, 9 aa, synthetic construct
GGGGADKFI

SEQ ID NO: 26427 - protein, 9 aa, synthetic construct
GGRGKDALS

SEQ ID NO: 26428 - protein, 9 aa, synthetic construct
GGRGKDAFV

SEQ ID NO: 26429 - protein, 9 aa, synthetic construct
GGRGIDYLR

SEQ ID NO: 26430 - protein, 9 aa, synthetic construct
GGAGRDEII

SEQ ID NO: 26431 - protein, 9 aa, synthetic construct
GGAGRDEIS

SEQ ID NO: 26432 - protein, 9 aa, synthetic construct
GGRGIDTYY

SEQ ID NO: 26433 - protein, 9 aa, synthetic construct
GGRGIDTLI

SEQ ID NO: 26434 - protein, 9 aa, synthetic construct
GGAGRDELN

SEQ ID NO: 26435 - protein, 9 aa, synthetic construct
GGRGKDRLD

SEQ ID NO: 26436 - protein, 9 aa, synthetic construct
GGAGRDAYV

SEQ ID NO: 26437 - protein, 9 aa, synthetic construct
GGRGGDSMK

SEQ ID NO: 26438 - protein, 9 aa, synthetic construct
GGRGKDSFV

SEQ ID NO: 26439 - protein, 9 aa, synthetic construct
GGAGQDYIT

SEQ ID NO: 26440 - protein, 9 aa, synthetic construct
GGAGQDYLV

SEQ ID NO: 26441 - protein, 9 aa, synthetic construct
GGAGQDYLY

SEQ ID NO: 26442 - protein, 9 aa, synthetic construct
GGAGQDYMD

SEQ ID NO: 26443 - protein, 9 aa, synthetic construct
GGAGQDYVR

SEQ ID NO: 26444 - protein, 9 aa, synthetic construct
GGRGLDTLS

SEQ ID NO: 26445 - protein, 9 aa, synthetic construct
GGEGHDIIT

SEQ ID NO: 26446 - protein, 9 aa, synthetic construct
GGGGADIIY

SEQ ID NO: 26447 - protein, 9 aa, synthetic construct
GGAGRDAIL

SEQ ID NO: 26448 - protein, 9 aa, synthetic construct
GGGGADILF

SEQ ID NO: 26449 - protein, 9 aa, synthetic construct
GGGGADILH

SEQ ID NO: 26450 - protein, 9 aa, synthetic construct
GGRGKDYID

SEQ ID NO: 26451 - protein, 9 aa, synthetic construct
GGAGRDALI

SEQ ID NO: 26452 - protein, 9 aa, synthetic construct
GGGGADILL

SEQ ID NO: 26453 - protein, 9 aa, synthetic construct
GGRGKDVLV

SEQ ID NO: 26454 - protein, 9 aa, synthetic construct
GGRGKDVLN

SEQ ID NO: 26455 - protein, 9 aa, synthetic construct
GGRGKDVLK

SEQ ID NO: 26456 - protein, 9 aa, synthetic construct
GGRGKDVLI

SEQ ID NO: 26457 - protein, 9 aa, synthetic construct
GGRGKDVFK

SEQ ID NO: 26458 - protein, 9 aa, synthetic construct
GGRGKDTYY

SEQ ID NO: 26459 - protein, 9 aa, synthetic construct
GGRGKDTYV

SEQ ID NO: 26460 - protein, 9 aa, synthetic construct
GGRGKDTLT

SEQ ID NO: 26461 - protein, 9 aa, synthetic construct
GGRGKDTLK

SEQ ID NO: 26462 - protein, 9 aa, synthetic construct
GGAGRDELQ

SEQ ID NO: 26463 - protein, 9 aa, synthetic construct
GGRGIDTAS

SEQ ID NO: 26464 - protein, 9 aa, synthetic construct
GGAGRDELY

SEQ ID NO: 26465 - protein, 9 aa, synthetic construct
GGAGRDEMD

SEQ ID NO: 26466 - protein, 9 aa, synthetic construct
GGAGRDHLA

SEQ ID NO: 26467 - protein, 9 aa, synthetic construct
GGRGHDILF

SEQ ID NO: 26468 - protein, 9 aa, synthetic construct
GGAGRDHLD

SEQ ID NO: 26469 - protein, 9 aa, synthetic construct
GGGGADKMS

SEQ ID NO: 26470 - protein, 9 aa, synthetic construct
GGGGADKMW

SEQ ID NO: 26471 - protein, 9 aa, synthetic construct
GGAGRDHLS

SEQ ID NO: 26472 - protein, 9 aa, synthetic construct
GGEGHDALD

SEQ ID NO: 26473 - protein, 9 aa, synthetic construct
GGRGGDYLI

SEQ ID NO: 26474 - protein, 9 aa, synthetic construct
GGRGGDWVV

SEQ ID NO: 26475 - protein, 9 aa, synthetic construct
GGAGRDHME

SEQ ID NO: 26476 - protein, 9 aa, synthetic construct
GGRGGDVMR

SEQ ID NO: 26477 - protein, 9 aa, synthetic construct
GGAGRDHVD

SEQ ID NO: 26478 - protein, 9 aa, synthetic construct
GGRGGDVLQ

SEQ ID NO: 26479 - protein, 9 aa, synthetic construct
GGAGRDHVH

SEQ ID NO: 26480 - protein, 9 aa, synthetic construct
GGAGRDHVV

SEQ ID NO: 26481 - protein, 9 aa, synthetic construct
GGRGGDTVF

SEQ ID NO: 26482 - protein, 9 aa, synthetic construct
GGRGGDTMS

SEQ ID NO: 26483 - protein, 9 aa, synthetic construct
GGRGGDTLA

SEQ ID NO: 26484 - protein, 9 aa, synthetic construct
GGAGRDIAS

SEQ ID NO: 26485 - protein, 9 aa, synthetic construct
GGAGRDIFI

SEQ ID NO: 26486 - protein, 9 aa, synthetic construct
GGRGGDTIE

SEQ ID NO: 26487 - protein, 9 aa, synthetic construct
GGRGGDSVT

SEQ ID NO: 26488 - protein, 9 aa, synthetic construct
GGAGRDIFR

SEQ ID NO: 26489 - protein, 9 aa, synthetic construct
GGAGRDHFV

SEQ ID NO: 26490 - protein, 9 aa, synthetic construct
GGRGHDKLF

SEQ ID NO: 26491 - protein, 9 aa, synthetic construct
GGRGHDLLK

SEQ ID NO: 26492 - protein, 9 aa, synthetic construct
GGRGHDTLT

SEQ ID NO: 26493 - protein, 9 aa, synthetic construct
GGGGADKIN

SEQ ID NO: 26494 - protein, 9 aa, synthetic construct
GGRGIDRIA

SEQ ID NO: 26495 - protein, 9 aa, synthetic construct
GGGGADKIT

SEQ ID NO: 26496 - protein, 9 aa, synthetic construct
GGGGADKIW

SEQ ID NO: 26497 - protein, 9 aa, synthetic construct
GGAGRDFFY

SEQ ID NO: 26498 - protein, 9 aa, synthetic construct
GGRGHDYLR

SEQ ID NO: 26499 - protein, 9 aa, synthetic construct
GGGGADKLD

SEQ ID NO: 26500 - protein, 9 aa, synthetic construct
GGAGRDFIL

SEQ ID NO: 26501 - protein, 9 aa, synthetic construct
GGRGHDVLY

SEQ ID NO: 26502 - protein, 9 aa, synthetic construct
GGGGADKLF

SEQ ID NO: 26503 - protein, 9 aa, synthetic construct
GGAGRDFMN

SEQ ID NO: 26504 - protein, 9 aa, synthetic construct
GGAGRDGLS

SEQ ID NO: 26505 - protein, 9 aa, synthetic construct
GGAGRDFVD

SEQ ID NO: 26506 - protein, 9 aa, synthetic construct
GGRGHDTID

SEQ ID NO: 26507 - protein, 9 aa, synthetic construct
GGRGHDSVE

SEQ ID NO: 26508 - protein, 9 aa, synthetic construct
GGAGRDFVS

SEQ ID NO: 26509 - protein, 9 aa, synthetic construct
GGRGHDSLT

SEQ ID NO: 26510 - protein, 9 aa, synthetic construct
GGGGADKLM

SEQ ID NO: 26511 - protein, 9 aa, synthetic construct
GGRGHDRLN

SEQ ID NO: 26512 - protein, 9 aa, synthetic construct
GGAGRDGFI

SEQ ID NO: 26513 - protein, 9 aa, synthetic construct
GGGGADKLQ

SEQ ID NO: 26514 - protein, 9 aa, synthetic construct
GGGGADKLV

SEQ ID NO: 26515 - protein, 9 aa, synthetic construct
GGGGADMLN

SEQ ID NO: 26516 - protein, 9 aa, synthetic construct
GGRGDDMLT

SEQ ID NO: 26517 - protein, 9 aa, synthetic construct
GGAGRDQLI

SEQ ID NO: 26518 - protein, 9 aa, synthetic construct
GGRGADILS

SEQ ID NO: 26519 - protein, 9 aa, synthetic construct
GGRGADILD

SEQ ID NO: 26520 - protein, 9 aa, synthetic construct
GGRGADHLD

SEQ ID NO: 26521 - protein, 9 aa, synthetic construct
GGRGADGLL

SEQ ID NO: 26522 - protein, 9 aa, synthetic construct
GGRGADEMH

SEQ ID NO: 26523 - protein, 9 aa, synthetic construct
GGRGADELY

SEQ ID NO: 26524 - protein, 9 aa, synthetic construct
GGRGADELT

SEQ ID NO: 26525 - protein, 9 aa, synthetic construct
GGRGADELI

SEQ ID NO: 26526 - protein, 9 aa, synthetic construct
GGAGRDVIF

SEQ ID NO: 26527 - protein, 9 aa, synthetic construct
GGRGADDLY

SEQ ID NO: 26528 - protein, 9 aa, synthetic construct
GGAGRDVIH

SEQ ID NO: 26529 - protein, 9 aa, synthetic construct
GGAGRDVII

SEQ ID NO: 26530 - protein, 9 aa, synthetic construct
GGAGRDVIS

SEQ ID NO: 26531 - protein, 9 aa, synthetic construct
GGRGADALA

SEQ ID NO: 26532 - protein, 9 aa, synthetic construct
GGAGRDVLM

SEQ ID NO: 26533 - protein, 9 aa, synthetic construct
GGQGYDLIF

SEQ ID NO: 26534 - protein, 9 aa, synthetic construct
GGQGYDILH

SEQ ID NO: 26535 - protein, 9 aa, synthetic construct
GGQGWDRMG

SEQ ID NO: 26536 - protein, 9 aa, synthetic construct
GGQGWDELH

SEQ ID NO: 26537 - protein, 9 aa, synthetic construct
GGQGWDEFV

SEQ ID NO: 26538 - protein, 9 aa, synthetic construct
GGAGRDVMD

SEQ ID NO: 26539 - protein, 9 aa, synthetic construct
GGAGRDVMH

SEQ ID NO: 26540 - protein, 9 aa, synthetic construct
GGAGRDVMK

SEQ ID NO: 26541 - protein, 9 aa, synthetic construct
GGQGVDVLF

SEQ ID NO: 26542 - protein, 9 aa, synthetic construct
GGEGGDTFA

SEQ ID NO: 26543 - protein, 9 aa, synthetic construct
GGRGADIMA

SEQ ID NO: 26544 - protein, 9 aa, synthetic construct
GGRGADRMN

SEQ ID NO: 26545 - protein, 9 aa, synthetic construct
GGEGGDTFV

SEQ ID NO: 26546 - protein, 9 aa, synthetic construct
GGRGADRLL

SEQ ID NO: 26547 - protein, 9 aa, synthetic construct
GGRGADRIL

SEQ ID NO: 26548 - protein, 9 aa, synthetic construct
GGRGADRAF

SEQ ID NO: 26549 - protein, 9 aa, synthetic construct
GGAGRDTMI

SEQ ID NO: 26550 - protein, 9 aa, synthetic construct
GGAGRDTMQ

SEQ ID NO: 26551 - protein, 9 aa, synthetic construct
GGRGADQFV

SEQ ID NO: 26552 - protein, 9 aa, synthetic construct
GGAGRDTMS

SEQ ID NO: 26553 - protein, 9 aa, synthetic construct
GGRGADNLN

SEQ ID NO: 26554 - protein, 9 aa, synthetic construct
GGRGADNFV

SEQ ID NO: 26555 - protein, 9 aa, synthetic construct
GGRGADMLT

SEQ ID NO: 26556 - protein, 9 aa, synthetic construct
GGAGRDTVD

SEQ ID NO: 26557 - protein, 9 aa, synthetic construct
GGAGRDTVG

SEQ ID NO: 26558 - protein, 9 aa, synthetic construct
GGRGADLMR

SEQ ID NO: 26559 - protein, 9 aa, synthetic construct
GGGGADQMT

SEQ ID NO: 26560 - protein, 9 aa, synthetic construct
GGRGADLLV

SEQ ID NO: 26561 - protein, 9 aa, synthetic construct
GGRGADLLT

SEQ ID NO: 26562 - protein, 9 aa, synthetic construct
GGRGADLLI

SEQ ID NO: 26563 - protein, 9 aa, synthetic construct
GGRGADLIS

SEQ ID NO: 26564 - protein, 9 aa, synthetic construct
GGAGRDTVV

SEQ ID NO: 26565 - protein, 9 aa, synthetic construct
GGAGRDTVY

SEQ ID NO: 26566 - protein, 9 aa, synthetic construct
GGRGADKLF

SEQ ID NO: 26567 - protein, 9 aa, synthetic construct
GGGGADQYV

SEQ ID NO: 26568 - protein, 9 aa, synthetic construct
GGAGRDVAR

SEQ ID NO: 26569 - protein, 9 aa, synthetic construct
GGAGRDVMN

SEQ ID NO: 26570 - protein, 9 aa, synthetic construct
GGAGRDVMV

SEQ ID NO: 26571 - protein, 9 aa, synthetic construct
GGQGVDTLQ

SEQ ID NO: 26572 - protein, 9 aa, synthetic construct
GGAGRDVVM

SEQ ID NO: 26573 - protein, 9 aa, synthetic construct
GGAGSDAIK

SEQ ID NO: 26574 - protein, 9 aa, synthetic construct
GGQGTDFVR

SEQ ID NO: 26575 - protein, 9 aa, synthetic construct
GGAGSDALA

SEQ ID NO: 26576 - protein, 9 aa, synthetic construct
GGQGSDVMY

SEQ ID NO: 26577 - protein, 9 aa, synthetic construct
GGAGSDALT

SEQ ID NO: 26578 - protein, 9 aa, synthetic construct
GGQGSDVLI

SEQ ID NO: 26579 - protein, 9 aa, synthetic construct
GGAGSDAMT

SEQ ID NO: 26580 - protein, 9 aa, synthetic construct
GGQGSDVID

SEQ ID NO: 26581 - protein, 9 aa, synthetic construct
GGEGGDSID

SEQ ID NO: 26582 - protein, 9 aa, synthetic construct
GGAGSDAYA

SEQ ID NO: 26583 - protein, 9 aa, synthetic construct
GGAGSDAYY

SEQ ID NO: 26584 - protein, 9 aa, synthetic construct
GGQGSDTLW

SEQ ID NO: 26585 - protein, 9 aa, synthetic construct
GGQGSDTLK

SEQ ID NO: 26586 - protein, 9 aa, synthetic construct
GGQGSDTLI

SEQ ID NO: 26587 - protein, 9 aa, synthetic construct
GGQGSDTLA

SEQ ID NO: 26588 - protein, 9 aa, synthetic construct
GGQGSDTIN

SEQ ID NO: 26589 - protein, 9 aa, synthetic construct
GGAGSDDIL

SEQ ID NO: 26590 - protein, 9 aa, synthetic construct
GGQGSDSVR

SEQ ID NO: 26591 - protein, 9 aa, synthetic construct
GGQGSDSLS

SEQ ID NO: 26592 - protein, 9 aa, synthetic construct
GGAGSDDLH

SEQ ID NO: 26593 - protein, 9 aa, synthetic construct
GGQGSDSIS

SEQ ID NO: 26594 - protein, 9 aa, synthetic construct
GGQGSDSID

SEQ ID NO: 26595 - protein, 9 aa, synthetic construct
GGQGSDRME

SEQ ID NO: 26596 - protein, 9 aa, synthetic construct
GGQGTDILT

SEQ ID NO: 26597 - protein, 9 aa, synthetic construct
GGAGSDAID

SEQ ID NO: 26598 - protein, 9 aa, synthetic construct
GGQGTDSLD

SEQ ID NO: 26599 - protein, 9 aa, synthetic construct
GGQGTDYLD

SEQ ID NO: 26600 - protein, 9 aa, synthetic construct
GGQGVDTIV

SEQ ID NO: 26601 - protein, 9 aa, synthetic construct
GGEGGDSLF

SEQ ID NO: 26602 - protein, 9 aa, synthetic construct
GGEGGDSLE

SEQ ID NO: 26603 - protein, 9 aa, synthetic construct
GGAGRDWAL

SEQ ID NO: 26604 - protein, 9 aa, synthetic construct
GGEGGDSLD

SEQ ID NO: 26605 - protein, 9 aa, synthetic construct
GGGGADRIV

SEQ ID NO: 26606 - protein, 9 aa, synthetic construct
GGAGRDWIM

SEQ ID NO: 26607 - protein, 9 aa, synthetic construct
GGGGADRIW

SEQ ID NO: 26608 - protein, 9 aa, synthetic construct
GGAGRDWLA

SEQ ID NO: 26609 - protein, 9 aa, synthetic construct
GGAGRDWLF

SEQ ID NO: 26610 - protein, 9 aa, synthetic construct
GGAGRDYFH

SEQ ID NO: 26611 - protein, 9 aa, synthetic construct
GGQGTDSLF

SEQ ID NO: 26612 - protein, 9 aa, synthetic construct
GGGGADRLG

SEQ ID NO: 26613 - protein, 9 aa, synthetic construct
GGAGRDYIY

SEQ ID NO: 26614 - protein, 9 aa, synthetic construct
GGQGTDTMY

SEQ ID NO: 26615 - protein, 9 aa, synthetic construct
GGQGTDTLT

SEQ ID NO: 26616 - protein, 9 aa, synthetic construct
GGAGRDYLE

SEQ ID NO: 26617 - protein, 9 aa, synthetic construct
GGGGADRLH

SEQ ID NO: 26618 - protein, 9 aa, synthetic construct
GGQGTDTIY

SEQ ID NO: 26619 - protein, 9 aa, synthetic construct
GGQGTDTIS

SEQ ID NO: 26620 - protein, 9 aa, synthetic construct
GGQGTDTID

SEQ ID NO: 26621 - protein, 9 aa, synthetic construct
GGAGRDYMS

SEQ ID NO: 26622 - protein, 9 aa, synthetic construct
GGRGADRLV

SEQ ID NO: 26623 - protein, 9 aa, synthetic construct
GGRGADRMT

SEQ ID NO: 26624 - protein, 9 aa, synthetic construct
GGGGADMLS

SEQ ID NO: 26625 - protein, 9 aa, synthetic construct
GGAGRDRLC

SEQ ID NO: 26626 - protein, 9 aa, synthetic construct
GGRGDDIIH

SEQ ID NO: 26627 - protein, 9 aa, synthetic construct
GGAGRDRLH

SEQ ID NO: 26628 - protein, 9 aa, synthetic construct
GGRGDDIFL

SEQ ID NO: 26629 - protein, 9 aa, synthetic construct
GGRGDDHLR

SEQ ID NO: 26630 - protein, 9 aa, synthetic construct
GGRGDDHLQ

SEQ ID NO: 26631 - protein, 9 aa, synthetic construct
GGAGRDRLR

SEQ ID NO: 26632 - protein, 9 aa, synthetic construct
GGRGDDHLK

SEQ ID NO: 26633 - protein, 9 aa, synthetic construct
GGRGDDHLF

SEQ ID NO: 26634 - protein, 9 aa, synthetic construct
GGRGDDHLD

SEQ ID NO: 26635 - protein, 9 aa, synthetic construct
GGRGDDHID

SEQ ID NO: 26636 - protein, 9 aa, synthetic construct
GGRGDDGLT

SEQ ID NO: 26637 - protein, 9 aa, synthetic construct
GGAGRDRLW

SEQ ID NO: 26638 - protein, 9 aa, synthetic construct
GGAGRDRMA

SEQ ID NO: 26639 - protein, 9 aa, synthetic construct
GGAGRDRMD

SEQ ID NO: 26640 - protein, 9 aa, synthetic construct
GGRGDDFMN

SEQ ID NO: 26641 - protein, 9 aa, synthetic construct
GGRGDDFMD

SEQ ID NO: 26642 - protein, 9 aa, synthetic construct
GGAGRDRML

SEQ ID NO: 26643 - protein, 9 aa, synthetic construct
GGRGDDFLV

SEQ ID NO: 26644 - protein, 9 aa, synthetic construct
GGAGRDRMV

SEQ ID NO: 26645 - protein, 9 aa, synthetic construct
GGAGRDRVA

SEQ ID NO: 26646 - protein, 9 aa, synthetic construct
GGRGDDFLD

SEQ ID NO: 26647 - protein, 9 aa, synthetic construct
GGGGADNLT

SEQ ID NO: 26648 - protein, 9 aa, synthetic construct
GGRGDDFII

SEQ ID NO: 26649 - protein, 9 aa, synthetic construct
GGQGDDALD

SEQ ID NO: 26650 - protein, 9 aa, synthetic construct
GGRGDDILV

SEQ ID NO: 26651 - protein, 9 aa, synthetic construct
GGAGRDTLM

SEQ ID NO: 26652 - protein, 9 aa, synthetic construct
GGRGDDILW

SEQ ID NO: 26653 - protein, 9 aa, synthetic construct
GGGGADMLT

SEQ ID NO: 26654 - protein, 9 aa, synthetic construct
GGAGRDQLR

SEQ ID NO: 26655 - protein, 9 aa, synthetic construct
GGAGRDQLT

SEQ ID NO: 26656 - protein, 9 aa, synthetic construct
GGRGDDLYL

SEQ ID NO: 26657 - protein, 9 aa, synthetic construct
GGGGADMVG

SEQ ID NO: 26658 - protein, 9 aa, synthetic construct
GGRGDDLVI

SEQ ID NO: 26659 - protein, 9 aa, synthetic construct
GGRGDDLVF

SEQ ID NO: 26660 - protein, 9 aa, synthetic construct
GGAGRDRAD

SEQ ID NO: 26661 - protein, 9 aa, synthetic construct
GGGGADNFI

SEQ ID NO: 26662 - protein, 9 aa, synthetic construct
GGRGDDLMN

SEQ ID NO: 26663 - protein, 9 aa, synthetic construct
GGAGRDRAS

SEQ ID NO: 26664 - protein, 9 aa, synthetic construct
GGRGDDLLK

SEQ ID NO: 26665 - protein, 9 aa, synthetic construct
GGAGRDRFT

SEQ ID NO: 26666 - protein, 9 aa, synthetic construct
GGRGDDLIV

SEQ ID NO: 26667 - protein, 9 aa, synthetic construct
GGRGDDLIL

SEQ ID NO: 26668 - protein, 9 aa, synthetic construct
GGGGADNID

SEQ ID NO: 26669 - protein, 9 aa, synthetic construct
GGRGDDLIE

SEQ ID NO: 26670 - protein, 9 aa, synthetic construct
GGGGADNIK

SEQ ID NO: 26671 - protein, 9 aa, synthetic construct
GGAGRDRIL

SEQ ID NO: 26672 - protein, 9 aa, synthetic construct
GGRGDDKID

SEQ ID NO: 26673 - protein, 9 aa, synthetic construct
GGAGRDRIV

SEQ ID NO: 26674 - protein, 9 aa, synthetic construct
GGRGDDIVR

SEQ ID NO: 26675 - protein, 9 aa, synthetic construct
GGRGDDIVE

SEQ ID NO: 26676 - protein, 9 aa, synthetic construct
GGAGRDRVH

SEQ ID NO: 26677 - protein, 9 aa, synthetic construct
GGRGDDFID

SEQ ID NO: 26678 - protein, 9 aa, synthetic construct
GGRGDDFAS

SEQ ID NO: 26679 - protein, 9 aa, synthetic construct
GGRGDDEVL

SEQ ID NO: 26680 - protein, 9 aa, synthetic construct
GGRGADVIQ

SEQ ID NO: 26681 - protein, 9 aa, synthetic construct
GGRGADVIH

SEQ ID NO: 26682 - protein, 9 aa, synthetic construct
GGRGADVID

SEQ ID NO: 26683 - protein, 9 aa, synthetic construct
GGAGRDTFE

SEQ ID NO: 26684 - protein, 9 aa, synthetic construct
GGRGADTYE

SEQ ID NO: 26685 - protein, 9 aa, synthetic construct
GGEGGDTIL

SEQ ID NO: 26686 - protein, 9 aa, synthetic construct
GGRGADTVK

SEQ ID NO: 26687 - protein, 9 aa, synthetic construct
GGRGADTMT

SEQ ID NO: 26688 - protein, 9 aa, synthetic construct
GGRGADTMS

SEQ ID NO: 26689 - protein, 9 aa, synthetic construct
GGGGADQLQ

SEQ ID NO: 26690 - protein, 9 aa, synthetic construct
GGRGADTMA

SEQ ID NO: 26691 - protein, 9 aa, synthetic construct
GGRGADTLK

SEQ ID NO: 26692 - protein, 9 aa, synthetic construct
GGRGADTLH

SEQ ID NO: 26693 - protein, 9 aa, synthetic construct
GGAGRDTIK

SEQ ID NO: 26694 - protein, 9 aa, synthetic construct
GGAGRDTIN

SEQ ID NO: 26695 - protein, 9 aa, synthetic construct
GGRGADTIE

SEQ ID NO: 26696 - protein, 9 aa, synthetic construct
GGAGRDTIR

SEQ ID NO: 26697 - protein, 9 aa, synthetic construct
GGAGRDTIT

SEQ ID NO: 26698 - protein, 9 aa, synthetic construct
GGRGADTFI

SEQ ID NO: 26699 - protein, 9 aa, synthetic construct
GGAGRDTIV

SEQ ID NO: 26700 - protein, 9 aa, synthetic construct
GGRGADTAS

SEQ ID NO: 26701 - protein, 9 aa, synthetic construct
GGRGADSLY

SEQ ID NO: 26702 - protein, 9 aa, synthetic construct
GGAGRDTLH

SEQ ID NO: 26703 - protein, 9 aa, synthetic construct
GGRGADVLR

SEQ ID NO: 26704 - protein, 9 aa, synthetic construct
GGEGGDTIN

SEQ ID NO: 26705 - protein, 9 aa, synthetic construct
GGAGRDTAE

SEQ ID NO: 26706 - protein, 9 aa, synthetic construct
GGRGDDALW

SEQ ID NO: 26707 - protein, 9 aa, synthetic construct
GGAGRDSAW

SEQ ID NO: 26708 - protein, 9 aa, synthetic construct
GGGGADNMN

SEQ ID NO: 26709 - protein, 9 aa, synthetic construct
GGAGRDSID

SEQ ID NO: 26710 - protein, 9 aa, synthetic construct
GGRGDDEIF

SEQ ID NO: 26711 - protein, 9 aa, synthetic construct
GGRGDDEID

SEQ ID NO: 26712 - protein, 9 aa, synthetic construct
GGRGDDDLR

SEQ ID NO: 26713 - protein, 9 aa, synthetic construct
GGRGDDDLH

SEQ ID NO: 26714 - protein, 9 aa, synthetic construct
GGRGDDDLG

SEQ ID NO: 26715 - protein, 9 aa, synthetic construct
GGAGRDSLA

SEQ ID NO: 26716 - protein, 9 aa, synthetic construct
GGRGDDDLD

SEQ ID NO: 26717 - protein, 9 aa, synthetic construct
GGAGRDSLM

SEQ ID NO: 26718 - protein, 9 aa, synthetic construct
GGGGADQLD

SEQ ID NO: 26719 - protein, 9 aa, synthetic construct
GGRGDDALN

SEQ ID NO: 26720 - protein, 9 aa, synthetic construct
GGRGDDALL

SEQ ID NO: 26721 - protein, 9 aa, synthetic construct
GGAGRDSMT

SEQ ID NO: 26722 - protein, 9 aa, synthetic construct
GGRGADYLS

SEQ ID NO: 26723 - protein, 9 aa, synthetic construct
GGRGADYLN

SEQ ID NO: 26724 - protein, 9 aa, synthetic construct
GGGGADQFR

SEQ ID NO: 26725 - protein, 9 aa, synthetic construct
GGRGADYLE

SEQ ID NO: 26726 - protein, 9 aa, synthetic construct
GGAGRDSVN

SEQ ID NO: 26727 - protein, 9 aa, synthetic construct
GGRGADWLD

SEQ ID NO: 26728 - protein, 9 aa, synthetic construct
GGGGADQIS

SEQ ID NO: 26729 - protein, 9 aa, synthetic construct
GGAGQDYIN

SEQ ID NO: 26730 - protein, 9 aa, synthetic construct
GGRGMDTLT

SEQ ID NO: 26731 - protein, 9 aa, synthetic construct
GGQGSDQLQ

SEQ ID NO: 26732 - protein, 9 aa, synthetic construct
GGRGSDTLF

SEQ ID NO: 26733 - protein, 9 aa, synthetic construct
GGRGSDTIL

SEQ ID NO: 26734 - protein, 9 aa, synthetic construct
GGAGPDDFI

SEQ ID NO: 26735 - protein, 9 aa, synthetic construct
GGRGSDTID

SEQ ID NO: 26736 - protein, 9 aa, synthetic construct
GGAGPDFLV

SEQ ID NO: 26737 - protein, 9 aa, synthetic construct
GGFGVDTLI

SEQ ID NO: 26738 - protein, 9 aa, synthetic construct
GGRGSDSLT

SEQ ID NO: 26739 - protein, 9 aa, synthetic construct
GGEGHDTMV

SEQ ID NO: 26740 - protein, 9 aa, synthetic construct
GGAGPDLLI

SEQ ID NO: 26741 - protein, 9 aa, synthetic construct
GGAGPDLLN

SEQ ID NO: 26742 - protein, 9 aa, synthetic construct
GGAGPDLLV

SEQ ID NO: 26743 - protein, 9 aa, synthetic construct
GGRGSDRLN

SEQ ID NO: 26744 - protein, 9 aa, synthetic construct
GGAGPDMLF

SEQ ID NO: 26745 - protein, 9 aa, synthetic construct
GGAGPDQLN

SEQ ID NO: 26746 - protein, 9 aa, synthetic construct
GGRGSDRIN

SEQ ID NO: 26747 - protein, 9 aa, synthetic construct
GGFGXDSIL

SEQ ID NO: 26748 - protein, 9 aa, synthetic construct
GGRGSDRFS

SEQ ID NO: 26749 - protein, 9 aa, synthetic construct
GGRGSDQMF

SEQ ID NO: 26750 - protein, 9 aa, synthetic construct
GGRGSDQLL

SEQ ID NO: 26751 - protein, 9 aa, synthetic construct
GGAGPDRFV

SEQ ID NO: 26752 - protein, 9 aa, synthetic construct
GGEGHDTLS

SEQ ID NO: 26753 - protein, 9 aa, synthetic construct
GGEGHDTLR

SEQ ID NO: 26754 - protein, 9 aa, synthetic construct
GGRGSDMII

SEQ ID NO: 26755 - protein, 9 aa, synthetic construct
GGEGHDTLN

SEQ ID NO: 26756 - protein, 9 aa, synthetic construct
GGRGSDTLA

SEQ ID NO: 26757 - protein, 9 aa, synthetic construct
GGRGSDTLL

SEQ ID NO: 26758 - protein, 9 aa, synthetic construct
GGAGPDRLY

SEQ ID NO: 26759 - protein, 9 aa, synthetic construct
GGRGSDTLR

SEQ ID NO: 26760 - protein, 9 aa, synthetic construct
GGRGTDTLH

SEQ ID NO: 26761 - protein, 9 aa, synthetic construct
GGRGTDSLD

SEQ ID NO: 26762 - protein, 9 aa, synthetic construct
GGAGNDYLG

SEQ ID NO: 26763 - protein, 9 aa, synthetic construct
GGRGTDMLY

SEQ ID NO: 26764 - protein, 9 aa, synthetic construct
GGRGTDMAL

SEQ ID NO: 26765 - protein, 9 aa, synthetic construct
GGRGTDLLR

SEQ ID NO: 26766 - protein, 9 aa, synthetic construct
GGRGTDIMS

SEQ ID NO: 26767 - protein, 9 aa, synthetic construct
GGRGTDAYY

SEQ ID NO: 26768 - protein, 9 aa, synthetic construct
GGFGVDKMI

SEQ ID NO: 26769 - protein, 9 aa, synthetic construct
GGAGNDYMK

SEQ ID NO: 26770 - protein, 9 aa, synthetic construct
GGAGNDYMM

SEQ ID NO: 26771 - protein, 9 aa, synthetic construct
GGAGNDYMR

SEQ ID NO: 26772 - protein, 9 aa, synthetic construct
GGRGSDYLD

SEQ ID NO: 26773 - protein, 9 aa, synthetic construct
GGRGSDYLA

SEQ ID NO: 26774 - protein, 9 aa, synthetic construct
GGRGSDWLD

SEQ ID NO: 26775 - protein, 9 aa, synthetic construct
GGAGNDYVH

SEQ ID NO: 26776 - protein, 9 aa, synthetic construct
GGRGSDVLT

SEQ ID NO: 26777 - protein, 9 aa, synthetic construct
GGAGNDYVS

SEQ ID NO: 26778 - protein, 9 aa, synthetic construct
GGAGNDYVT

SEQ ID NO: 26779 - protein, 9 aa, synthetic construct
GGRGSDVIS

SEQ ID NO: 26780 - protein, 9 aa, synthetic construct
GGRGSDVID

SEQ ID NO: 26781 - protein, 9 aa, synthetic construct
GGFGVDNLF

SEQ ID NO: 26782 - protein, 9 aa, synthetic construct
GGAGPDAFV

SEQ ID NO: 26783 - protein, 9 aa, synthetic construct
GGRGSDLYL

SEQ ID NO: 26784 - protein, 9 aa, synthetic construct
GGFGYDQMV

SEQ ID NO: 26785 - protein, 9 aa, synthetic construct
GGRGMDVVF

SEQ ID NO: 26786 - protein, 9 aa, synthetic construct
GGRGSDALE

SEQ ID NO: 26787 - protein, 9 aa, synthetic construct
GGGGADAFY

SEQ ID NO: 26788 - protein, 9 aa, synthetic construct
GGRGRDYLL

SEQ ID NO: 26789 - protein, 9 aa, synthetic construct
GGRGRDYIS

SEQ ID NO: 26790 - protein, 9 aa, synthetic construct
GGAGPDWLA

SEQ ID NO: 26791 - protein, 9 aa, synthetic construct
GGAGPDWLR

SEQ ID NO: 26792 - protein, 9 aa, synthetic construct
GGRGRDVYE

SEQ ID NO: 26793 - protein, 9 aa, synthetic construct
GGAGQDAFR

SEQ ID NO: 26794 - protein, 9 aa, synthetic construct
GGGGADAID

SEQ ID NO: 26795 - protein, 9 aa, synthetic construct
GGRGRDVLT

SEQ ID NO: 26796 - protein, 9 aa, synthetic construct
GGRGRDVLF

SEQ ID NO: 26797 - protein, 9 aa, synthetic construct
GGGGADALA

SEQ ID NO: 26798 - protein, 9 aa, synthetic construct
GGAGQDALD

SEQ ID NO: 26799 - protein, 9 aa, synthetic construct
GGRGRDTVT

SEQ ID NO: 26800 - protein, 9 aa, synthetic construct
GGRGRDTVR

SEQ ID NO: 26801 - protein, 9 aa, synthetic construct
GGRGRDTVQ

SEQ ID NO: 26802 - protein, 9 aa, synthetic construct
GGRGRDTLT

SEQ ID NO: 26803 - protein, 9 aa, synthetic construct
GGRGRDTLR

SEQ ID NO: 26804 - protein, 9 aa, synthetic construct
GGAGQDAVF

SEQ ID NO: 26805 - protein, 9 aa, synthetic construct
GGAGQDDIS

SEQ ID NO: 26806 - protein, 9 aa, synthetic construct
GGRGRDTIY

SEQ ID NO: 26807 - protein, 9 aa, synthetic construct
GGRGRDTIV

SEQ ID NO: 26808 - protein, 9 aa, synthetic construct
GGRGRDTIN

SEQ ID NO: 26809 - protein, 9 aa, synthetic construct
GGRGRDTIK

SEQ ID NO: 26810 - protein, 9 aa, synthetic construct
GGRGSDAFV

SEQ ID NO: 26811 - protein, 9 aa, synthetic construct
GGRGSDALF

SEQ ID NO: 26812 - protein, 9 aa, synthetic construct
GGAGPDRMY

SEQ ID NO: 26813 - protein, 9 aa, synthetic construct
GGRGSDALT

SEQ ID NO: 26814 - protein, 9 aa, synthetic construct
GGRGSDLLI

SEQ ID NO: 26815 - protein, 9 aa, synthetic construct
GGFGYDRLH

SEQ ID NO: 26816 - protein, 9 aa, synthetic construct
GGAGPDTFF

SEQ ID NO: 26817 - protein, 9 aa, synthetic construct
GGRGSDLIL

SEQ ID NO: 26818 - protein, 9 aa, synthetic construct
GGAGPDTFL

SEQ ID NO: 26819 - protein, 9 aa, synthetic construct
GGRGSDKLN

SEQ ID NO: 26820 - protein, 9 aa, synthetic construct
GGAGPDTIV

SEQ ID NO: 26821 - protein, 9 aa, synthetic construct
GGAGPDTLD

SEQ ID NO: 26822 - protein, 9 aa, synthetic construct
GGRGSDILS

SEQ ID NO: 26823 - protein, 9 aa, synthetic construct
GGAGPDTLH

SEQ ID NO: 26824 - protein, 9 aa, synthetic construct
GGAGPDTLL

SEQ ID NO: 26825 - protein, 9 aa, synthetic construct
GGFGYDRMN

SEQ ID NO: 26826 - protein, 9 aa, synthetic construct
GGRGSDIII

SEQ ID NO: 26827 - protein, 9 aa, synthetic construct
GGAGPDTLN

SEQ ID NO: 26828 - protein, 9 aa, synthetic construct
GGRGSDHLH

SEQ ID NO: 26829 - protein, 9 aa, synthetic construct
GGFGYDSLD

SEQ ID NO: 26830 - protein, 9 aa, synthetic construct
GGFGYDTLD

SEQ ID NO: 26831 - protein, 9 aa, synthetic construct
GGRGSDFIR

SEQ ID NO: 26832 - protein, 9 aa, synthetic construct
GGGGADAFL

SEQ ID NO: 26833 - protein, 9 aa, synthetic construct
GGEGHDTLA

SEQ ID NO: 26834 - protein, 9 aa, synthetic construct
GGGGADAFQ

SEQ ID NO: 26835 - protein, 9 aa, synthetic construct
GGRGSDAVI

SEQ ID NO: 26836 - protein, 9 aa, synthetic construct
GGRGSDALY

SEQ ID NO: 26837 - protein, 9 aa, synthetic construct
GGRGTDTLL

SEQ ID NO: 26838 - protein, 9 aa, synthetic construct
GGAGNDYIQ

SEQ ID NO: 26839 - protein, 9 aa, synthetic construct
GGAGNDYIM

SEQ ID NO: 26840 - protein, 9 aa, synthetic construct
GGSGADIML

SEQ ID NO: 26841 - protein, 9 aa, synthetic construct
GGSGADIIY

SEQ ID NO: 26842 - protein, 9 aa, synthetic construct
GGSGADIIS

SEQ ID NO: 26843 - protein, 9 aa, synthetic construct
GGSGADIIN

SEQ ID NO: 26844 - protein, 9 aa, synthetic construct
GGAGNDVMF

SEQ ID NO: 26845 - protein, 9 aa, synthetic construct
GGSGADIIA

SEQ ID NO: 26846 - protein, 9 aa, synthetic construct
GGSGADIFD

SEQ ID NO: 26847 - protein, 9 aa, synthetic construct
GGSGADIAS

SEQ ID NO: 26848 - protein, 9 aa, synthetic construct
GGSGADIAD

SEQ ID NO: 26849 - protein, 9 aa, synthetic construct
GGSGADIAA

SEQ ID NO: 26850 - protein, 9 aa, synthetic construct
GGSGADHMV

SEQ ID NO: 26851 - protein, 9 aa, synthetic construct
GGSGADHMK

SEQ ID NO: 26852 - protein, 9 aa, synthetic construct
GGSGADHMI

SEQ ID NO: 26853 - protein, 9 aa, synthetic construct
GGSGADHLD

SEQ ID NO: 26854 - protein, 9 aa, synthetic construct
GGSGADGFV

SEQ ID NO: 26855 - protein, 9 aa, synthetic construct
GGSGADFLV

SEQ ID NO: 26856 - protein, 9 aa, synthetic construct
GGAGNDVVV

SEQ ID NO: 26857 - protein, 9 aa, synthetic construct
GGSGADFLF

SEQ ID NO: 26858 - protein, 9 aa, synthetic construct
GGEGIDFVQ

SEQ ID NO: 26859 - protein, 9 aa, synthetic construct
GGSGADFID

SEQ ID NO: 26860 - protein, 9 aa, synthetic construct
GGSGADEVF

SEQ ID NO: 26861 - protein, 9 aa, synthetic construct
GGSGADEMT

SEQ ID NO: 26862 - protein, 9 aa, synthetic construct
GGSGADEMR

SEQ ID NO: 26863 - protein, 9 aa, synthetic construct
GGSGADELS

SEQ ID NO: 26864 - protein, 9 aa, synthetic construct
GGSGADILK

SEQ ID NO: 26865 - protein, 9 aa, synthetic construct
GGSGADKFD

SEQ ID NO: 26866 - protein, 9 aa, synthetic construct
GGRGTDVLL

SEQ ID NO: 26867 - protein, 9 aa, synthetic construct
GGSGADKFL

SEQ ID NO: 26868 - protein, 9 aa, synthetic construct
GGAGNDVFN

SEQ ID NO: 26869 - protein, 9 aa, synthetic construct
GGSGADLVF

SEQ ID NO: 26870 - protein, 9 aa, synthetic construct
GGAGNDVFQ

SEQ ID NO: 26871 - protein, 9 aa, synthetic construct
GGSGADLMN

SEQ ID NO: 26872 - protein, 9 aa, synthetic construct
GGSGADLMI

SEQ ID NO: 26873 - protein, 9 aa, synthetic construct
GGSGADLLY

SEQ ID NO: 26874 - protein, 9 aa, synthetic construct
GGSGADLLT

SEQ ID NO: 26875 - protein, 9 aa, synthetic construct
GGSGADLLQ

SEQ ID NO: 26876 - protein, 9 aa, synthetic construct
GGSGADLLM

SEQ ID NO: 26877 - protein, 9 aa, synthetic construct
GGSGADLIS

SEQ ID NO: 26878 - protein, 9 aa, synthetic construct
GGSGADLIR

SEQ ID NO: 26879 - protein, 9 aa, synthetic construct
GGSGADLIN

SEQ ID NO: 26880 - protein, 9 aa, synthetic construct
GGSGADLIH

SEQ ID NO: 26881 - protein, 9 aa, synthetic construct
GGSGADLIF

SEQ ID NO: 26882 - protein, 9 aa, synthetic construct
GGSGADLFK

SEQ ID NO: 26883 - protein, 9 aa, synthetic construct
GGAGNDVIK

SEQ ID NO: 26884 - protein, 9 aa, synthetic construct
GGAGNDVIM

SEQ ID NO: 26885 - protein, 9 aa, synthetic construct
GGSGADKMY

SEQ ID NO: 26886 - protein, 9 aa, synthetic construct
GGSGADKMT

SEQ ID NO: 26887 - protein, 9 aa, synthetic construct
GGSGADKLV

SEQ ID NO: 26888 - protein, 9 aa, synthetic construct
GGSGADKLK

SEQ ID NO: 26889 - protein, 9 aa, synthetic construct
GGSGADKLE

SEQ ID NO: 26890 - protein, 9 aa, synthetic construct
GGFGTDHMD

SEQ ID NO: 26891 - protein, 9 aa, synthetic construct
GGSGADELH

SEQ ID NO: 26892 - protein, 9 aa, synthetic construct
GGSGADEIY

SEQ ID NO: 26893 - protein, 9 aa, synthetic construct
GGSGADEIG

SEQ ID NO: 26894 - protein, 9 aa, synthetic construct
GGSGADEFV

SEQ ID NO: 26895 - protein, 9 aa, synthetic construct
GGFGTDYLH

SEQ ID NO: 26896 - protein, 9 aa, synthetic construct
GGRGWDSAH

SEQ ID NO: 26897 - protein, 9 aa, synthetic construct
GGRGVDTMV

SEQ ID NO: 26898 - protein, 9 aa, synthetic construct
GGAGNDWME

SEQ ID NO: 26899 - protein, 9 aa, synthetic construct
GGAGNDWMH

SEQ ID NO: 26900 - protein, 9 aa, synthetic construct
GGRGVDTLD

SEQ ID NO: 26901 - protein, 9 aa, synthetic construct
GGAGNDWMW

SEQ ID NO: 26902 - protein, 9 aa, synthetic construct
GGAGNDWVA

SEQ ID NO: 26903 - protein, 9 aa, synthetic construct
GGAGNDWVD

SEQ ID NO: 26904 - protein, 9 aa, synthetic construct
GGFGVDDLD

SEQ ID NO: 26905 - protein, 9 aa, synthetic construct
GGFGVDELI

SEQ ID NO: 26906 - protein, 9 aa, synthetic construct
GGFGVDEVI

SEQ ID NO: 26907 - protein, 9 aa, synthetic construct
GGAGNDWVW

SEQ ID NO: 26908 - protein, 9 aa, synthetic construct
GGAGNDWVY

SEQ ID NO: 26909 - protein, 9 aa, synthetic construct
GGAGNDWYF

SEQ ID NO: 26910 - protein, 9 aa, synthetic construct
GGRGVDRLI

SEQ ID NO: 26911 - protein, 9 aa, synthetic construct
GGEGHDWLE

SEQ ID NO: 26912 - protein, 9 aa, synthetic construct
GGAGNDYAH

SEQ ID NO: 26913 - protein, 9 aa, synthetic construct
GGRGVDKLH

SEQ ID NO: 26914 - protein, 9 aa, synthetic construct
GGRGVDALY

SEQ ID NO: 26915 - protein, 9 aa, synthetic construct
GGAGNDYIG

SEQ ID NO: 26916 - protein, 9 aa, synthetic construct
GGRGVDALH

SEQ ID NO: 26917 - protein, 9 aa, synthetic construct
GGRGTDVVT

SEQ ID NO: 26918 - protein, 9 aa, synthetic construct
GGRGWDVLL

SEQ ID NO: 26919 - protein, 9 aa, synthetic construct
GGRGYDELY

SEQ ID NO: 26920 - protein, 9 aa, synthetic construct
GGRGYDILN

SEQ ID NO: 26921 - protein, 9 aa, synthetic construct
GGSGADAVY

SEQ ID NO: 26922 - protein, 9 aa, synthetic construct
GGSGADEFI

SEQ ID NO: 26923 - protein, 9 aa, synthetic construct
GGSGADDMR

SEQ ID NO: 26924 - protein, 9 aa, synthetic construct
GGSGADDLR

SEQ ID NO: 26925 - protein, 9 aa, synthetic construct
GGSGADDLQ

SEQ ID NO: 26926 - protein, 9 aa, synthetic construct
GGSGADDLG

SEQ ID NO: 26927 - protein, 9 aa, synthetic construct
GGSGADDIT

SEQ ID NO: 26928 - protein, 9 aa, synthetic construct
GGFGTDTVI

SEQ ID NO: 26929 - protein, 9 aa, synthetic construct
GGSGADDID

SEQ ID NO: 26930 - protein, 9 aa, synthetic construct
GGAGNDWIN

SEQ ID NO: 26931 - protein, 9 aa, synthetic construct
GGAGNDWIQ

SEQ ID NO: 26932 - protein, 9 aa, synthetic construct
GGAGNDWIR

SEQ ID NO: 26933 - protein, 9 aa, synthetic construct
GGAGNDWLK

SEQ ID NO: 26934 - protein, 9 aa, synthetic construct
GGSGADAMA

SEQ ID NO: 26935 - protein, 9 aa, synthetic construct
GGSGADALY

SEQ ID NO: 26936 - protein, 9 aa, synthetic construct
GGSGADALS

SEQ ID NO: 26937 - protein, 9 aa, synthetic construct
GGFGTDVLM

SEQ ID NO: 26938 - protein, 9 aa, synthetic construct
GGAGNDWIY

SEQ ID NO: 26939 - protein, 9 aa, synthetic construct
GGSGADALK

SEQ ID NO: 26940 - protein, 9 aa, synthetic construct
GGSGADAIF

SEQ ID NO: 26941 - protein, 9 aa, synthetic construct
GGSGADAFI

SEQ ID NO: 26942 - protein, 9 aa, synthetic construct
GGRGYDTLM

SEQ ID NO: 26943 - protein, 9 aa, synthetic construct
GGRGYDLIR

SEQ ID NO: 26944 - protein, 9 aa, synthetic construct
GGGGADALI

SEQ ID NO: 26945 - protein, 9 aa, synthetic construct
GGRGRDTID

SEQ ID NO: 26946 - protein, 9 aa, synthetic construct
GGRGRDTFI

SEQ ID NO: 26947 - protein, 9 aa, synthetic construct
GGAGQDSFV

SEQ ID NO: 26948 - protein, 9 aa, synthetic construct
GGRGNDRML

SEQ ID NO: 26949 - protein, 9 aa, synthetic construct
GGRGNDRLW

SEQ ID NO: 26950 - protein, 9 aa, synthetic construct
GGGGADGLA

SEQ ID NO: 26951 - protein, 9 aa, synthetic construct
GGAGQDSIS

SEQ ID NO: 26952 - protein, 9 aa, synthetic construct
GGAGQDSIY

SEQ ID NO: 26953 - protein, 9 aa, synthetic construct
GGGGADGLD

SEQ ID NO: 26954 - protein, 9 aa, synthetic construct
GGRGNDRIF

SEQ ID NO: 26955 - protein, 9 aa, synthetic construct
GGEGHDLLS

SEQ ID NO: 26956 - protein, 9 aa, synthetic construct
GGGGADGLN

SEQ ID NO: 26957 - protein, 9 aa, synthetic construct
GGEGHDLLE

SEQ ID NO: 26958 - protein, 9 aa, synthetic construct
GGAGQDSMY

SEQ ID NO: 26959 - protein, 9 aa, synthetic construct
GGRGNDNLT

SEQ ID NO: 26960 - protein, 9 aa, synthetic construct
GGGGADHLD

SEQ ID NO: 26961 - protein, 9 aa, synthetic construct
GGEGHDKLV

SEQ ID NO: 26962 - protein, 9 aa, synthetic construct
GGEGHDKLI

SEQ ID NO: 26963 - protein, 9 aa, synthetic construct
GGAGQDTFA

SEQ ID NO: 26964 - protein, 9 aa, synthetic construct
GGRGNDMLY

SEQ ID NO: 26965 - protein, 9 aa, synthetic construct
GGRGNDMLS

SEQ ID NO: 26966 - protein, 9 aa, synthetic construct
GGRGNDMLI

SEQ ID NO: 26967 - protein, 9 aa, synthetic construct
GGAGQDTFK

SEQ ID NO: 26968 - protein, 9 aa, synthetic construct
GGRGNDMID

SEQ ID NO: 26969 - protein, 9 aa, synthetic construct
GGGGADHLL

SEQ ID NO: 26970 - protein, 9 aa, synthetic construct
GGRGNDLYI

SEQ ID NO: 26971 - protein, 9 aa, synthetic construct
GGAGQDSID

SEQ ID NO: 26972 - protein, 9 aa, synthetic construct
GGRGNDRVS

SEQ ID NO: 26973 - protein, 9 aa, synthetic construct
GGAGQDQLS

SEQ ID NO: 26974 - protein, 9 aa, synthetic construct
GGGGADGIG

SEQ ID NO: 26975 - protein, 9 aa, synthetic construct
GGGGADFLH

SEQ ID NO: 26976 - protein, 9 aa, synthetic construct
GGRGNDTVD

SEQ ID NO: 26977 - protein, 9 aa, synthetic construct
GGGGADFLI

SEQ ID NO: 26978 - protein, 9 aa, synthetic construct
GGRGNDTLM

SEQ ID NO: 26979 - protein, 9 aa, synthetic construct
GGRGNDTIM

SEQ ID NO: 26980 - protein, 9 aa, synthetic construct
GGRGNDTII

SEQ ID NO: 26981 - protein, 9 aa, synthetic construct
GGRGNDTFY

SEQ ID NO: 26982 - protein, 9 aa, synthetic construct
GGAGQDRID

SEQ ID NO: 26983 - protein, 9 aa, synthetic construct
GGRGNDTAY

SEQ ID NO: 26984 - protein, 9 aa, synthetic construct
GGGGADFLV

SEQ ID NO: 26985 - protein, 9 aa, synthetic construct
GGRGNDTAR

SEQ ID NO: 26986 - protein, 9 aa, synthetic construct
GGRGNDSYI

SEQ ID NO: 26987 - protein, 9 aa, synthetic construct
GGAGQDRLI

SEQ ID NO: 26988 - protein, 9 aa, synthetic construct
GGRGNDSMA

SEQ ID NO: 26989 - protein, 9 aa, synthetic construct
GGGGADFML

SEQ ID NO: 26990 - protein, 9 aa, synthetic construct
GGRGNDSLN

SEQ ID NO: 26991 - protein, 9 aa, synthetic construct
GGGGADFVN

SEQ ID NO: 26992 - protein, 9 aa, synthetic construct
GGRGNDSLK

SEQ ID NO: 26993 - protein, 9 aa, synthetic construct
GGRGNDSIW

SEQ ID NO: 26994 - protein, 9 aa, synthetic construct
GGAGQDRLS

SEQ ID NO: 26995 - protein, 9 aa, synthetic construct
GGRGNDSIF

SEQ ID NO: 26996 - protein, 9 aa, synthetic construct
GGRGNDSIE

SEQ ID NO: 26997 - protein, 9 aa, synthetic construct
GGAGQDRLY

SEQ ID NO: 26998 - protein, 9 aa, synthetic construct
GGRGNDLVH

SEQ ID NO: 26999 - protein, 9 aa, synthetic construct
GGRGNDLMS

SEQ ID NO: 27000 - protein, 9 aa, synthetic construct
GGRGNDLMN

SEQ ID NO: 27001 - protein, 9 aa, synthetic construct
GGAGQDTIF

SEQ ID NO: 27002 - protein, 9 aa, synthetic construct
GGRGNDIID

SEQ ID NO: 27003 - protein, 9 aa, synthetic construct
GGAGQDTML

SEQ ID NO: 27004 - protein, 9 aa, synthetic construct
GGAGQDTVL

SEQ ID NO: 27005 - protein, 9 aa, synthetic construct
GGRGNDHIR

SEQ ID NO: 27006 - protein, 9 aa, synthetic construct
GGAGQDTYA

SEQ ID NO: 27007 - protein, 9 aa, synthetic construct
GGAGQDTYL

SEQ ID NO: 27008 - protein, 9 aa, synthetic construct
GGRGNDGLA

SEQ ID NO: 27009 - protein, 9 aa, synthetic construct
GGRGNDGIS

SEQ ID NO: 27010 - protein, 9 aa, synthetic construct
GGRGNDFLV

SEQ ID NO: 27011 - protein, 9 aa, synthetic construct
GGRGNDFLI

SEQ ID NO: 27012 - protein, 9 aa, synthetic construct
GGEGHDILV

SEQ ID NO: 27013 - protein, 9 aa, synthetic construct
GGRGNDELF

SEQ ID NO: 27014 - protein, 9 aa, synthetic construct
GGGGADIFF

SEQ ID NO: 27015 - protein, 9 aa, synthetic construct
GGAGQDVIR

SEQ ID NO: 27016 - protein, 9 aa, synthetic construct
GGRGNDEIF

SEQ ID NO: 27017 - protein, 9 aa, synthetic construct
GGRGNDDLR

SEQ ID NO: 27018 - protein, 9 aa, synthetic construct
GGRGNDDLF

SEQ ID NO: 27019 - protein, 9 aa, synthetic construct
GGAGQDVLR

SEQ ID NO: 27020 - protein, 9 aa, synthetic construct
GGGGADIFN

SEQ ID NO: 27021 - protein, 9 aa, synthetic construct
GGAGQDVVT

SEQ ID NO: 27022 - protein, 9 aa, synthetic construct
GGAGQDVVY

SEQ ID NO: 27023 - protein, 9 aa, synthetic construct
GGRGNDAIS

SEQ ID NO: 27024 - protein, 9 aa, synthetic construct
GGAGQDWLR

SEQ ID NO: 27025 - protein, 9 aa, synthetic construct
GGAGQDTMF

SEQ ID NO: 27026 - protein, 9 aa, synthetic construct
GGGGADHME

SEQ ID NO: 27027 - protein, 9 aa, synthetic construct
GGRGNDIIN

SEQ ID NO: 27028 - protein, 9 aa, synthetic construct
GGRGNDKMF

SEQ ID NO: 27029 - protein, 9 aa, synthetic construct
GGAGQDTIH

SEQ ID NO: 27030 - protein, 9 aa, synthetic construct
GGAGQDTII

SEQ ID NO: 27031 - protein, 9 aa, synthetic construct
GGAGQDTIN

SEQ ID NO: 27032 - protein, 9 aa, synthetic construct
GGRGNDLIY

SEQ ID NO: 27033 - protein, 9 aa, synthetic construct
GGGGADHLT

SEQ ID NO: 27034 - protein, 9 aa, synthetic construct
GGRGNDLIR

SEQ ID NO: 27035 - protein, 9 aa, synthetic construct
GGAGQDTIT

SEQ ID NO: 27036 - protein, 9 aa, synthetic construct
GGAGQDTIY

SEQ ID NO: 27037 - protein, 9 aa, synthetic construct
GGRGNDLAH

SEQ ID NO: 27038 - protein, 9 aa, synthetic construct
GGRGNDKMY

SEQ ID NO: 27039 - protein, 9 aa, synthetic construct
GGRGNDKLW

SEQ ID NO: 27040 - protein, 9 aa, synthetic construct
GGRGNDIIS

SEQ ID NO: 27041 - protein, 9 aa, synthetic construct
GGAGQDTLH

SEQ ID NO: 27042 - protein, 9 aa, synthetic construct
GGRGNDKLK

SEQ ID NO: 27043 - protein, 9 aa, synthetic construct
GGRGNDKID

SEQ ID NO: 27044 - protein, 9 aa, synthetic construct
GGRGNDIYY

SEQ ID NO: 27045 - protein, 9 aa, synthetic construct
GGAGQDTLM

SEQ ID NO: 27046 - protein, 9 aa, synthetic construct
GGRGNDIVY

SEQ ID NO: 27047 - protein, 9 aa, synthetic construct
GGRGNDIVR

SEQ ID NO: 27048 - protein, 9 aa, synthetic construct
GGRGNDIVL

SEQ ID NO: 27049 - protein, 9 aa, synthetic construct
GGRGNDIMI

SEQ ID NO: 27050 - protein, 9 aa, synthetic construct
GGRGNDILA

SEQ ID NO: 27051 - protein, 9 aa, synthetic construct
GGRGNDTYH

SEQ ID NO: 27052 - protein, 9 aa, synthetic construct
GGRGNDVAL

SEQ ID NO: 27053 - protein, 9 aa, synthetic construct
GGAGQDDLY

SEQ ID NO: 27054 - protein, 9 aa, synthetic construct
GGAGQDHLY

SEQ ID NO: 27055 - protein, 9 aa, synthetic construct
GGEGHDSLT

SEQ ID NO: 27056 - protein, 9 aa, synthetic construct
GGAGQDIFL

SEQ ID NO: 27057 - protein, 9 aa, synthetic construct
GGAGQDIIR

SEQ ID NO: 27058 - protein, 9 aa, synthetic construct
GGRGRDKLD

SEQ ID NO: 27059 - protein, 9 aa, synthetic construct
GGRGRDILN

SEQ ID NO: 27060 - protein, 9 aa, synthetic construct
GGGGADDID

SEQ ID NO: 27061 - protein, 9 aa, synthetic construct
GGRGRDILI

SEQ ID NO: 27062 - protein, 9 aa, synthetic construct
GGRGRDIFV

SEQ ID NO: 27063 - protein, 9 aa, synthetic construct
GGEGHDSLL

SEQ ID NO: 27064 - protein, 9 aa, synthetic construct
GGRGRDFLW

SEQ ID NO: 27065 - protein, 9 aa, synthetic construct
GGRGRDFLV

SEQ ID NO: 27066 - protein, 9 aa, synthetic construct
GGEGHDSLI

SEQ ID NO: 27067 - protein, 9 aa, synthetic construct
GGAGQDILR

SEQ ID NO: 27068 - protein, 9 aa, synthetic construct
GGAGQDILS

SEQ ID NO: 27069 - protein, 9 aa, synthetic construct
GGRGRDELH

SEQ ID NO: 27070 - protein, 9 aa, synthetic construct
GGRGRDELF

SEQ ID NO: 27071 - protein, 9 aa, synthetic construct
GGAGQDIVT

SEQ ID NO: 27072 - protein, 9 aa, synthetic construct
GGRGRDDIS

SEQ ID NO: 27073 - protein, 9 aa, synthetic construct
GGRGRDDFQ

SEQ ID NO: 27074 - protein, 9 aa, synthetic construct
GGGGADDLD

SEQ ID NO: 27075 - protein, 9 aa, synthetic construct
GGAGQDKIS

SEQ ID NO: 27076 - protein, 9 aa, synthetic construct
GGRGRDALD

SEQ ID NO: 27077 - protein, 9 aa, synthetic construct
GGAGQDKLD

SEQ ID NO: 27078 - protein, 9 aa, synthetic construct
GGAGQDIAK

SEQ ID NO: 27079 - protein, 9 aa, synthetic construct
GGRGRDLLM

SEQ ID NO: 27080 - protein, 9 aa, synthetic construct
GGRGNDVAS

SEQ ID NO: 27081 - protein, 9 aa, synthetic construct
GGRGRDLLS

SEQ ID NO: 27082 - protein, 9 aa, synthetic construct
GGGGADALL

SEQ ID NO: 27083 - protein, 9 aa, synthetic construct
GGGGADALR

SEQ ID NO: 27084 - protein, 9 aa, synthetic construct
GGRGRDSLD

SEQ ID NO: 27085 - protein, 9 aa, synthetic construct
GGAGQDELT

SEQ ID NO: 27086 - protein, 9 aa, synthetic construct
GGRGRDRMN

SEQ ID NO: 27087 - protein, 9 aa, synthetic construct
GGAGQDELW

SEQ ID NO: 27088 - protein, 9 aa, synthetic construct
GGGGADAMA

SEQ ID NO: 27089 - protein, 9 aa, synthetic construct
GGRGRDRLI

SEQ ID NO: 27090 - protein, 9 aa, synthetic construct
GGRGRDRLD

SEQ ID NO: 27091 - protein, 9 aa, synthetic construct
GGEGHDSMN

SEQ ID NO: 27092 - protein, 9 aa, synthetic construct
GGAGQDEYS

SEQ ID NO: 27093 - protein, 9 aa, synthetic construct
GGAGQDFAN

SEQ ID NO: 27094 - protein, 9 aa, synthetic construct
GGAGQDFFV

SEQ ID NO: 27095 - protein, 9 aa, synthetic construct
GGAGQDFIW

SEQ ID NO: 27096 - protein, 9 aa, synthetic construct
GGRGRDQMF

SEQ ID NO: 27097 - protein, 9 aa, synthetic construct
GGGGADAMI

SEQ ID NO: 27098 - protein, 9 aa, synthetic construct
GGRGRDQIE

SEQ ID NO: 27099 - protein, 9 aa, synthetic construct
GGAGQDFLQ

SEQ ID NO: 27100 - protein, 9 aa, synthetic construct
GGEGHDSLY

SEQ ID NO: 27101 - protein, 9 aa, synthetic construct
GGAGQDHAH

SEQ ID NO: 27102 - protein, 9 aa, synthetic construct
GGAGQDHIA

SEQ ID NO: 27103 - protein, 9 aa, synthetic construct
GGRGRDMLD

SEQ ID NO: 27104 - protein, 9 aa, synthetic construct
GGRGRDMIG

SEQ ID NO: 27105 - protein, 9 aa, synthetic construct
GGAGQDKLW

SEQ ID NO: 27106 - protein, 9 aa, synthetic construct
GGRGQDVLL

SEQ ID NO: 27107 - protein, 9 aa, synthetic construct
GGRGQDVLG

SEQ ID NO: 27108 - protein, 9 aa, synthetic construct
GGAGQDKVR

SEQ ID NO: 27109 - protein, 9 aa, synthetic construct
GGRGPDLLD

SEQ ID NO: 27110 - protein, 9 aa, synthetic construct
GGRGPDILR

SEQ ID NO: 27111 - protein, 9 aa, synthetic construct
GGGGADELK

SEQ ID NO: 27112 - protein, 9 aa, synthetic construct
GGRGNDYLR

SEQ ID NO: 27113 - protein, 9 aa, synthetic construct
GGRGNDYLN

SEQ ID NO: 27114 - protein, 9 aa, synthetic construct
GGRGNDYLK

SEQ ID NO: 27115 - protein, 9 aa, synthetic construct
GGRGNDWLV

SEQ ID NO: 27116 - protein, 9 aa, synthetic construct
GGAGQDNIG

SEQ ID NO: 27117 - protein, 9 aa, synthetic construct
GGAGQDNLE

SEQ ID NO: 27118 - protein, 9 aa, synthetic construct
GGRGNDVYY

SEQ ID NO: 27119 - protein, 9 aa, synthetic construct
GGRGNDVYT

SEQ ID NO: 27120 - protein, 9 aa, synthetic construct
GGRGNDVYH

SEQ ID NO: 27121 - protein, 9 aa, synthetic construct
GGRGNDVVE

SEQ ID NO: 27122 - protein, 9 aa, synthetic construct
GGAGQDNVA

SEQ ID NO: 27123 - protein, 9 aa, synthetic construct
GGRGNDVMI

SEQ ID NO: 27124 - protein, 9 aa, synthetic construct
GGGGADFID

SEQ ID NO: 27125 - protein, 9 aa, synthetic construct
GGRGNDVLH

SEQ ID NO: 27126 - protein, 9 aa, synthetic construct
GGAGQDQFR

SEQ ID NO: 27127 - protein, 9 aa, synthetic construct
GGGGADFIK

SEQ ID NO: 27128 - protein, 9 aa, synthetic construct
GGGGADFIN

SEQ ID NO: 27129 - protein, 9 aa, synthetic construct
GGGGADFIR

SEQ ID NO: 27130 - protein, 9 aa, synthetic construct
GGRGNDVIG

SEQ ID NO: 27131 - protein, 9 aa, synthetic construct
GGAGQDQLR

SEQ ID NO: 27132 - protein, 9 aa, synthetic construct
GGRGPDRFV

SEQ ID NO: 27133 - protein, 9 aa, synthetic construct
GGRGPDRIW

SEQ ID NO: 27134 - protein, 9 aa, synthetic construct
GGGGADELF

SEQ ID NO: 27135 - protein, 9 aa, synthetic construct
GGRGQDQLF

SEQ ID NO: 27136 - protein, 9 aa, synthetic construct
GGRGQDTVL

SEQ ID NO: 27137 - protein, 9 aa, synthetic construct
GGRGQDTLN

SEQ ID NO: 27138 - protein, 9 aa, synthetic construct
GGRGQDTLI

SEQ ID NO: 27139 - protein, 9 aa, synthetic construct
GGEGHDRLT

SEQ ID NO: 27140 - protein, 9 aa, synthetic construct
GGRGQDSIT

SEQ ID NO: 27141 - protein, 9 aa, synthetic construct
GGRGQDSFI

SEQ ID NO: 27142 - protein, 9 aa, synthetic construct
GGAGQDLLA

SEQ ID NO: 27143 - protein, 9 aa, synthetic construct
GGRGQDRLI

SEQ ID NO: 27144 - protein, 9 aa, synthetic construct
GGRGQDQLT

SEQ ID NO: 27145 - protein, 9 aa, synthetic construct
GGRGQDQLL

SEQ ID NO: 27146 - protein, 9 aa, synthetic construct
GGRGQDMLG

SEQ ID NO: 27147 - protein, 9 aa, synthetic construct
GGEGHDRIK

SEQ ID NO: 27148 - protein, 9 aa, synthetic construct
GGAGQDLLI

SEQ ID NO: 27149 - protein, 9 aa, synthetic construct
GGGGADEFT

SEQ ID NO: 27150 - protein, 9 aa, synthetic construct
GGRGQDLLK

SEQ ID NO: 27151 - protein, 9 aa, synthetic construct
GGRGQDLAV

SEQ ID NO: 27152 - protein, 9 aa, synthetic construct
GGAGQDLLN

SEQ ID NO: 27153 - protein, 9 aa, synthetic construct
GGRGQDILI

SEQ ID NO: 27154 - protein, 9 aa, synthetic construct
GGAGQDLLR

SEQ ID NO: 27155 - protein, 9 aa, synthetic construct
GGRGQDELY

SEQ ID NO: 27156 - protein, 9 aa, synthetic construct
GGGGADEFV

SEQ ID NO: 27157 - protein, 9 aa, synthetic construct
GGEGHDRLD

SEQ ID NO: 27158 - protein, 9 aa, synthetic construct
GGAGSDDLT

SEQ ID NO: 27159 - protein, 9 aa, synthetic construct
GGRGDDILH

SEQ ID NO: 27160 - protein, 9 aa, synthetic construct
GGQGSDNID

SEQ ID NO: 27161 - protein, 9 aa, synthetic construct
GGQGKDKIY

SEQ ID NO: 27162 - protein, 9 aa, synthetic construct
GGGGADVIA

SEQ ID NO: 27163 - protein, 9 aa, synthetic construct
GGQGLDNLF

SEQ ID NO: 27164 - protein, 9 aa, synthetic construct
GGQGLDLVY

SEQ ID NO: 27165 - protein, 9 aa, synthetic construct
GGQGLDGVF

SEQ ID NO: 27166 - protein, 9 aa, synthetic construct
GGQGKDYLN

SEQ ID NO: 27167 - protein, 9 aa, synthetic construct
GGQGKDVLY

SEQ ID NO: 27168 - protein, 9 aa, synthetic construct
GGAGSDRME

SEQ ID NO: 27169 - protein, 9 aa, synthetic construct
GGAGSDRMI

SEQ ID NO: 27170 - protein, 9 aa, synthetic construct
GGQGKDVFA

SEQ ID NO: 27171 - protein, 9 aa, synthetic construct
GGQGKDTYD

SEQ ID NO: 27172 - protein, 9 aa, synthetic construct
GGAGSDRVD

SEQ ID NO: 27173 - protein, 9 aa, synthetic construct
GGQGKDTLI

SEQ ID NO: 27174 - protein, 9 aa, synthetic construct
GGGGADVIF

SEQ ID NO: 27175 - protein, 9 aa, synthetic construct
GGGGADVIH

SEQ ID NO: 27176 - protein, 9 aa, synthetic construct
GGQGKDSYN

SEQ ID NO: 27177 - protein, 9 aa, synthetic construct
GGAGSDDVD

SEQ ID NO: 27178 - protein, 9 aa, synthetic construct
GGAGSDRYI

SEQ ID NO: 27179 - protein, 9 aa, synthetic construct
GGAGSDRYL

SEQ ID NO: 27180 - protein, 9 aa, synthetic construct
GGQGKDRLD

SEQ ID NO: 27181 - protein, 9 aa, synthetic construct
GGQGLDNVS

SEQ ID NO: 27182 - protein, 9 aa, synthetic construct
GGAGSDRLG

SEQ ID NO: 27183 - protein, 9 aa, synthetic construct
GGQGLDTLF

SEQ ID NO: 27184 - protein, 9 aa, synthetic construct
GGQGNDALD

SEQ ID NO: 27185 - protein, 9 aa, synthetic construct
GGGGADVFF

SEQ ID NO: 27186 - protein, 9 aa, synthetic construct
GGAGSDQLK

SEQ ID NO: 27187 - protein, 9 aa, synthetic construct
GGAGSDQLR

SEQ ID NO: 27188 - protein, 9 aa, synthetic construct
GGQGNDDIQ

SEQ ID NO: 27189 - protein, 9 aa, synthetic construct
GGQGNDAVS

SEQ ID NO: 27190 - protein, 9 aa, synthetic construct
GGQGNDAVH

SEQ ID NO: 27191 - protein, 9 aa, synthetic construct
GGGGADVFN

SEQ ID NO: 27192 - protein, 9 aa, synthetic construct
GGAGSDQYT

SEQ ID NO: 27193 - protein, 9 aa, synthetic construct
GGQGNDALA

SEQ ID NO: 27194 - protein, 9 aa, synthetic construct
GGAGSDRIR

SEQ ID NO: 27195 - protein, 9 aa, synthetic construct
GGAGSDRFA

SEQ ID NO: 27196 - protein, 9 aa, synthetic construct
GGQGMDTIY

SEQ ID NO: 27197 - protein, 9 aa, synthetic construct
GGAGSDRIF

SEQ ID NO: 27198 - protein, 9 aa, synthetic construct
GGAGSDRIK

SEQ ID NO: 27199 - protein, 9 aa, synthetic construct
GGQGLDTYI

SEQ ID NO: 27200 - protein, 9 aa, synthetic construct
GGAGSDRIL

SEQ ID NO: 27201 - protein, 9 aa, synthetic construct
GGAGSDRIN

SEQ ID NO: 27202 - protein, 9 aa, synthetic construct
GGQGLDTLS

SEQ ID NO: 27203 - protein, 9 aa, synthetic construct
GGGGADVIS

SEQ ID NO: 27204 - protein, 9 aa, synthetic construct
GGGGADVIY

SEQ ID NO: 27205 - protein, 9 aa, synthetic construct
GGQGGDSIS

SEQ ID NO: 27206 - protein, 9 aa, synthetic construct
GGQGKDIIL

SEQ ID NO: 27207 - protein, 9 aa, synthetic construct
GGQGHDTIT

SEQ ID NO: 27208 - protein, 9 aa, synthetic construct
GGQGHDTID

SEQ ID NO: 27209 - protein, 9 aa, synthetic construct
GGAGSDSMT

SEQ ID NO: 27210 - protein, 9 aa, synthetic construct
GGAGSDSMY

SEQ ID NO: 27211 - protein, 9 aa, synthetic construct
GGAGSDSVD

SEQ ID NO: 27212 - protein, 9 aa, synthetic construct
GGAGSDSVN

SEQ ID NO: 27213 - protein, 9 aa, synthetic construct
GGAGSDSVV

SEQ ID NO: 27214 - protein, 9 aa, synthetic construct
GGAGSDSYF

SEQ ID NO: 27215 - protein, 9 aa, synthetic construct
GGQGHDLIQ

SEQ ID NO: 27216 - protein, 9 aa, synthetic construct
GGGGADVML

SEQ ID NO: 27217 - protein, 9 aa, synthetic construct
GGAGSDTAG

SEQ ID NO: 27218 - protein, 9 aa, synthetic construct
GGAGSDTAR

SEQ ID NO: 27219 - protein, 9 aa, synthetic construct
GGQGHDEIS

SEQ ID NO: 27220 - protein, 9 aa, synthetic construct
GGQGHDDMG

SEQ ID NO: 27221 - protein, 9 aa, synthetic construct
GGAGSDTAY

SEQ ID NO: 27222 - protein, 9 aa, synthetic construct
GGQGGDWIE

SEQ ID NO: 27223 - protein, 9 aa, synthetic construct
GGQGGDVLD

SEQ ID NO: 27224 - protein, 9 aa, synthetic construct
GGAGSDTFQ

SEQ ID NO: 27225 - protein, 9 aa, synthetic construct
GGAGSDTIE

SEQ ID NO: 27226 - protein, 9 aa, synthetic construct
GGQGHDTIY

SEQ ID NO: 27227 - protein, 9 aa, synthetic construct
GGQGHDTLD

SEQ ID NO: 27228 - protein, 9 aa, synthetic construct
GGQGHDTLF

SEQ ID NO: 27229 - protein, 9 aa, synthetic construct
GGAGSDSLQ

SEQ ID NO: 27230 - protein, 9 aa, synthetic construct
GGAGSDSFQ

SEQ ID NO: 27231 - protein, 9 aa, synthetic construct
GGQGKDFIF

SEQ ID NO: 27232 - protein, 9 aa, synthetic construct
GGQGKDAIF

SEQ ID NO: 27233 - protein, 9 aa, synthetic construct
GGEGGDKLF

SEQ ID NO: 27234 - protein, 9 aa, synthetic construct
GGQGIDVLR

SEQ ID NO: 27235 - protein, 9 aa, synthetic construct
GGQGIDTLV

SEQ ID NO: 27236 - protein, 9 aa, synthetic construct
GGQGIDTIV

SEQ ID NO: 27237 - protein, 9 aa, synthetic construct
GGAGSDSLH

SEQ ID NO: 27238 - protein, 9 aa, synthetic construct
GGQGHDYID

SEQ ID NO: 27239 - protein, 9 aa, synthetic construct
GGQGHDTLN

SEQ ID NO: 27240 - protein, 9 aa, synthetic construct
GGQGHDVLR

SEQ ID NO: 27241 - protein, 9 aa, synthetic construct
GGQGHDVLQ

SEQ ID NO: 27242 - protein, 9 aa, synthetic construct
GGQGHDVLL

SEQ ID NO: 27243 - protein, 9 aa, synthetic construct
GGQGHDVLD

SEQ ID NO: 27244 - protein, 9 aa, synthetic construct
GGQGHDTYA

SEQ ID NO: 27245 - protein, 9 aa, synthetic construct
GGQGHDTMF

SEQ ID NO: 27246 - protein, 9 aa, synthetic construct
GGAGSDSML

SEQ ID NO: 27247 - protein, 9 aa, synthetic construct
GGQGHDTLR

SEQ ID NO: 27248 - protein, 9 aa, synthetic construct
GGQGNDEFL

SEQ ID NO: 27249 - protein, 9 aa, synthetic construct
GGAGSDQIM

SEQ ID NO: 27250 - protein, 9 aa, synthetic construct
GGEGGDLLA

SEQ ID NO: 27251 - protein, 9 aa, synthetic construct
GGQGNDELH

SEQ ID NO: 27252 - protein, 9 aa, synthetic construct
GGAGSDLMD

SEQ ID NO: 27253 - protein, 9 aa, synthetic construct
GGQGNDQIY

SEQ ID NO: 27254 - protein, 9 aa, synthetic construct
GGGGADTMD

SEQ ID NO: 27255 - protein, 9 aa, synthetic construct
GGQGNDPVF

SEQ ID NO: 27256 - protein, 9 aa, synthetic construct
GGEGGDNLV

SEQ ID NO: 27257 - protein, 9 aa, synthetic construct
GGEGGDNLT

SEQ ID NO: 27258 - protein, 9 aa, synthetic construct
GGQGNDNLV

SEQ ID NO: 27259 - protein, 9 aa, synthetic construct
GGQGNDNLS

SEQ ID NO: 27260 - protein, 9 aa, synthetic construct
GGGGADTMK

SEQ ID NO: 27261 - protein, 9 aa, synthetic construct
GGQGNDNIV

SEQ ID NO: 27262 - protein, 9 aa, synthetic construct
GGAGSDLYI

SEQ ID NO: 27263 - protein, 9 aa, synthetic construct
GGAGSDLYL

SEQ ID NO: 27264 - protein, 9 aa, synthetic construct
GGQGNDNID

SEQ ID NO: 27265 - protein, 9 aa, synthetic construct
GGQGNDMVN

SEQ ID NO: 27266 - protein, 9 aa, synthetic construct
GGAGSDMAS

SEQ ID NO: 27267 - protein, 9 aa, synthetic construct
GGAGSDMFV

SEQ ID NO: 27268 - protein, 9 aa, synthetic construct
GGQGNDLVY

SEQ ID NO: 27269 - protein, 9 aa, synthetic construct
GGQGNDLVR

SEQ ID NO: 27270 - protein, 9 aa, synthetic construct
GGQGNDLVQ

SEQ ID NO: 27271 - protein, 9 aa, synthetic construct
GGQGNDQLD

SEQ ID NO: 27272 - protein, 9 aa, synthetic construct
GGQGNDQLI

SEQ ID NO: 27273 - protein, 9 aa, synthetic construct
GGQGNDQLM

SEQ ID NO: 27274 - protein, 9 aa, synthetic construct
GGQGNDSLQ

SEQ ID NO: 27275 - protein, 9 aa, synthetic construct
GGQGNDTFV

SEQ ID NO: 27276 - protein, 9 aa, synthetic construct
GGQGNDTFI

SEQ ID NO: 27277 - protein, 9 aa, synthetic construct
GGQGNDTAS

SEQ ID NO: 27278 - protein, 9 aa, synthetic construct
GGAGSDLFR

SEQ ID NO: 27279 - protein, 9 aa, synthetic construct
GGAGSDLII

SEQ ID NO: 27280 - protein, 9 aa, synthetic construct
GGQGNDSVE

SEQ ID NO: 27281 - protein, 9 aa, synthetic construct
GGQGNDSLW

SEQ ID NO: 27282 - protein, 9 aa, synthetic construct
GGQGNDSLR

SEQ ID NO: 27283 - protein, 9 aa, synthetic construct
GGQGNDSLN

SEQ ID NO: 27284 - protein, 9 aa, synthetic construct
GGQGNDQLY

SEQ ID NO: 27285 - protein, 9 aa, synthetic construct
GGQGNDSLA

SEQ ID NO: 27286 - protein, 9 aa, synthetic construct
GGQGNDSIN

SEQ ID NO: 27287 - protein, 9 aa, synthetic construct
GGQGNDSFI

SEQ ID NO: 27288 - protein, 9 aa, synthetic construct
GGQGNDRMA

SEQ ID NO: 27289 - protein, 9 aa, synthetic construct
GGQGNDRLK

SEQ ID NO: 27290 - protein, 9 aa, synthetic construct
GGQGNDRII

SEQ ID NO: 27291 - protein, 9 aa, synthetic construct
GGQGNDRIE

SEQ ID NO: 27292 - protein, 9 aa, synthetic construct
GGQGNDQVF

SEQ ID NO: 27293 - protein, 9 aa, synthetic construct
GGQGNDLVN

SEQ ID NO: 27294 - protein, 9 aa, synthetic construct
GGGGADTMV

SEQ ID NO: 27295 - protein, 9 aa, synthetic construct
GGAGSDMLD

SEQ ID NO: 27296 - protein, 9 aa, synthetic construct
GGAGSDNVY

SEQ ID NO: 27297 - protein, 9 aa, synthetic construct
GGAGSDNLQ

SEQ ID NO: 27298 - protein, 9 aa, synthetic construct
GGAGSDNLS

SEQ ID NO: 27299 - protein, 9 aa, synthetic construct
GGQGNDHLN

SEQ ID NO: 27300 - protein, 9 aa, synthetic construct
GGQGNDHLL

SEQ ID NO: 27301 - protein, 9 aa, synthetic construct
GGQGNDHLD

SEQ ID NO: 27302 - protein, 9 aa, synthetic construct
GGQGNDHIK

SEQ ID NO: 27303 - protein, 9 aa, synthetic construct
GGGGADTVS

SEQ ID NO: 27304 - protein, 9 aa, synthetic construct
GGAGSDNVQ

SEQ ID NO: 27305 - protein, 9 aa, synthetic construct
GGGGADTYI

SEQ ID NO: 27306 - protein, 9 aa, synthetic construct
GGAGSDNLF

SEQ ID NO: 27307 - protein, 9 aa, synthetic construct
GGQGNDFLS

SEQ ID NO: 27308 - protein, 9 aa, synthetic construct
GGQGNDFIY

SEQ ID NO: 27309 - protein, 9 aa, synthetic construct
GGQGNDFIH

SEQ ID NO: 27310 - protein, 9 aa, synthetic construct
GGQGNDFID

SEQ ID NO: 27311 - protein, 9 aa, synthetic construct
GGQGNDEVY

SEQ ID NO: 27312 - protein, 9 aa, synthetic construct
GGGGADVFA

SEQ ID NO: 27313 - protein, 9 aa, synthetic construct
GGAGSDQIF

SEQ ID NO: 27314 - protein, 9 aa, synthetic construct
GGQGNDELI

SEQ ID NO: 27315 - protein, 9 aa, synthetic construct
GGAGSDNLN

SEQ ID NO: 27316 - protein, 9 aa, synthetic construct
GGQGNDIIN

SEQ ID NO: 27317 - protein, 9 aa, synthetic construct
GGQGNDLMF

SEQ ID NO: 27318 - protein, 9 aa, synthetic construct
GGQGNDKLV

SEQ ID NO: 27319 - protein, 9 aa, synthetic construct
GGQGNDLIT

SEQ ID NO: 27320 - protein, 9 aa, synthetic construct
GGQGNDLIS

SEQ ID NO: 27321 - protein, 9 aa, synthetic construct
GGQGNDLIQ

SEQ ID NO: 27322 - protein, 9 aa, synthetic construct
GGQGNDLIL

SEQ ID NO: 27323 - protein, 9 aa, synthetic construct
GGQGNDLII

SEQ ID NO: 27324 - protein, 9 aa, synthetic construct
GGQGNDLIH

SEQ ID NO: 27325 - protein, 9 aa, synthetic construct
GGAGSDMLS

SEQ ID NO: 27326 - protein, 9 aa, synthetic construct
GGQGNDLFN

SEQ ID NO: 27327 - protein, 9 aa, synthetic construct
GGQGNDKLT

SEQ ID NO: 27328 - protein, 9 aa, synthetic construct
GGQGNDIIT

SEQ ID NO: 27329 - protein, 9 aa, synthetic construct
GGAGSDMVS

SEQ ID NO: 27330 - protein, 9 aa, synthetic construct
GGQGNDKLA

SEQ ID NO: 27331 - protein, 9 aa, synthetic construct
GGAGSDNFV

SEQ ID NO: 27332 - protein, 9 aa, synthetic construct
GGQGNDIYV

SEQ ID NO: 27333 - protein, 9 aa, synthetic construct
GGQGNDIVY

SEQ ID NO: 27334 - protein, 9 aa, synthetic construct
GGQGNDIVS

SEQ ID NO: 27335 - protein, 9 aa, synthetic construct
GGQGNDIVR

SEQ ID NO: 27336 - protein, 9 aa, synthetic construct
GGGGADTVH

SEQ ID NO: 27337 - protein, 9 aa, synthetic construct
GGQGGDTIV

SEQ ID NO: 27338 - protein, 9 aa, synthetic construct
GGQGGDRLS

SEQ ID NO: 27339 - protein, 9 aa, synthetic construct
GGQGNDTIQ

SEQ ID NO: 27340 - protein, 9 aa, synthetic construct
GGQGDDKLL

SEQ ID NO: 27341 - protein, 9 aa, synthetic construct
GGGGDDAII

SEQ ID NO: 27342 - protein, 9 aa, synthetic construct
GGAGSDWMS

SEQ ID NO: 27343 - protein, 9 aa, synthetic construct
GGQGDDMIF

SEQ ID NO: 27344 - protein, 9 aa, synthetic construct
GGAGSDWMT

SEQ ID NO: 27345 - protein, 9 aa, synthetic construct
GGQGDDLVV

SEQ ID NO: 27346 - protein, 9 aa, synthetic construct
GGGGDDAIS

SEQ ID NO: 27347 - protein, 9 aa, synthetic construct
GGQGDDLVH

SEQ ID NO: 27348 - protein, 9 aa, synthetic construct
GGQGDDLMY

SEQ ID NO: 27349 - protein, 9 aa, synthetic construct
GGQGDDLMI

SEQ ID NO: 27350 - protein, 9 aa, synthetic construct
GGAGSDYFG

SEQ ID NO: 27351 - protein, 9 aa, synthetic construct
GGQGDDLLS

SEQ ID NO: 27352 - protein, 9 aa, synthetic construct
GGQGDDLLN

SEQ ID NO: 27353 - protein, 9 aa, synthetic construct
GGQGDDLLA

SEQ ID NO: 27354 - protein, 9 aa, synthetic construct
GGGGDDALF

SEQ ID NO: 27355 - protein, 9 aa, synthetic construct
GGGGDDALI

SEQ ID NO: 27356 - protein, 9 aa, synthetic construct
GGQGDDLII

SEQ ID NO: 27357 - protein, 9 aa, synthetic construct
GGQGDDLIE

SEQ ID NO: 27358 - protein, 9 aa, synthetic construct
GGQGDDLAH

SEQ ID NO: 27359 - protein, 9 aa, synthetic construct
GGAGSDYLL

SEQ ID NO: 27360 - protein, 9 aa, synthetic construct
GGQGDDMVR

SEQ ID NO: 27361 - protein, 9 aa, synthetic construct
GGAGSDWLM

SEQ ID NO: 27362 - protein, 9 aa, synthetic construct
GGQGDDNLM

SEQ ID NO: 27363 - protein, 9 aa, synthetic construct
GGGGDDAFV

SEQ ID NO: 27364 - protein, 9 aa, synthetic construct
GGQGDDRLV

SEQ ID NO: 27365 - protein, 9 aa, synthetic construct
GGQGDDRLR

SEQ ID NO: 27366 - protein, 9 aa, synthetic construct
GGQGDDRLH

SEQ ID NO: 27367 - protein, 9 aa, synthetic construct
GGQGDDRIY

SEQ ID NO: 27368 - protein, 9 aa, synthetic construct
GGQGDDRIS

SEQ ID NO: 27369 - protein, 9 aa, synthetic construct
GGAGSDVYY

SEQ ID NO: 27370 - protein, 9 aa, synthetic construct
GGAGSDWAD

SEQ ID NO: 27371 - protein, 9 aa, synthetic construct
GGQGDDQVF

SEQ ID NO: 27372 - protein, 9 aa, synthetic construct
GGGGDDAFY

SEQ ID NO: 27373 - protein, 9 aa, synthetic construct
GGQGDDNLR

SEQ ID NO: 27374 - protein, 9 aa, synthetic construct
GGQGDDQLW

SEQ ID NO: 27375 - protein, 9 aa, synthetic construct
GGQGDDQLS

SEQ ID NO: 27376 - protein, 9 aa, synthetic construct
GGAGSDWIE

SEQ ID NO: 27377 - protein, 9 aa, synthetic construct
GGEGFDYLD

SEQ ID NO: 27378 - protein, 9 aa, synthetic construct
GGQGDDQIT

SEQ ID NO: 27379 - protein, 9 aa, synthetic construct
GGQGDDQIS

SEQ ID NO: 27380 - protein, 9 aa, synthetic construct
GGAGSDWLE

SEQ ID NO: 27381 - protein, 9 aa, synthetic construct
GGAGSDWLF

SEQ ID NO: 27382 - protein, 9 aa, synthetic construct
GGQGDDKLR

SEQ ID NO: 27383 - protein, 9 aa, synthetic construct
GGQGDDKLD

SEQ ID NO: 27384 - protein, 9 aa, synthetic construct
GGQGGDRID

SEQ ID NO: 27385 - protein, 9 aa, synthetic construct
GGAGSDYLT

SEQ ID NO: 27386 - protein, 9 aa, synthetic construct
GGQGDDFYE

SEQ ID NO: 27387 - protein, 9 aa, synthetic construct
GGAGTDDLD

SEQ ID NO: 27388 - protein, 9 aa, synthetic construct
GGEGFDTVD

SEQ ID NO: 27389 - protein, 9 aa, synthetic construct
GGQGDDFVF

SEQ ID NO: 27390 - protein, 9 aa, synthetic construct
GGQGDDFLF

SEQ ID NO: 27391 - protein, 9 aa, synthetic construct
GGEGFDTLY

SEQ ID NO: 27392 - protein, 9 aa, synthetic construct
GGGGDDDLD

SEQ ID NO: 27393 - protein, 9 aa, synthetic construct
GGQGDDFID

SEQ ID NO: 27394 - protein, 9 aa, synthetic construct
GGAGTDEAH

SEQ ID NO: 27395 - protein, 9 aa, synthetic construct
GGEGFDTLT

SEQ ID NO: 27396 - protein, 9 aa, synthetic construct
GGAGTDEFN

SEQ ID NO: 27397 - protein, 9 aa, synthetic construct
GGQGDDEVH

SEQ ID NO: 27398 - protein, 9 aa, synthetic construct
GGGGDDDLR

SEQ ID NO: 27399 - protein, 9 aa, synthetic construct
GGQGDDDIY

SEQ ID NO: 27400 - protein, 9 aa, synthetic construct
GGAGTDFLD

SEQ ID NO: 27401 - protein, 9 aa, synthetic construct
GGQGDDDID

SEQ ID NO: 27402 - protein, 9 aa, synthetic construct
GGQGDDAYV

SEQ ID NO: 27403 - protein, 9 aa, synthetic construct
GGQGDDAVT

SEQ ID NO: 27404 - protein, 9 aa, synthetic construct
GGEGFDTLL

SEQ ID NO: 27405 - protein, 9 aa, synthetic construct
GGQGDDGLP

SEQ ID NO: 27406 - protein, 9 aa, synthetic construct
GGEGFDTYV

SEQ ID NO: 27407 - protein, 9 aa, synthetic construct
GGQGDDHID

SEQ ID NO: 27408 - protein, 9 aa, synthetic construct
GGQGDDILG

SEQ ID NO: 27409 - protein, 9 aa, synthetic construct
GGQGDDIYF

SEQ ID NO: 27410 - protein, 9 aa, synthetic construct
GGQGDDIVS

SEQ ID NO: 27411 - protein, 9 aa, synthetic construct
GGQGDDIVR

SEQ ID NO: 27412 - protein, 9 aa, synthetic construct
GGAGSDYMT

SEQ ID NO: 27413 - protein, 9 aa, synthetic construct
GGAGSDYVD

SEQ ID NO: 27414 - protein, 9 aa, synthetic construct
GGQGDDILW

SEQ ID NO: 27415 - protein, 9 aa, synthetic construct
GGQGDDILV

SEQ ID NO: 27416 - protein, 9 aa, synthetic construct
GGQGDDILL

SEQ ID NO: 27417 - protein, 9 aa, synthetic construct
GGQGDDILF

SEQ ID NO: 27418 - protein, 9 aa, synthetic construct
GGAGTDALT

SEQ ID NO: 27419 - protein, 9 aa, synthetic construct
GGAGSDYVV

SEQ ID NO: 27420 - protein, 9 aa, synthetic construct
GGGGDDALV

SEQ ID NO: 27421 - protein, 9 aa, synthetic construct
GGQGDDIIG

SEQ ID NO: 27422 - protein, 9 aa, synthetic construct
GGGGDDAMN

SEQ ID NO: 27423 - protein, 9 aa, synthetic construct
GGEGFDVLR

SEQ ID NO: 27424 - protein, 9 aa, synthetic construct
GGGGDDAYE

SEQ ID NO: 27425 - protein, 9 aa, synthetic construct
GGQGDDHLR

SEQ ID NO: 27426 - protein, 9 aa, synthetic construct
GGAGTDALN

SEQ ID NO: 27427 - protein, 9 aa, synthetic construct
GGQGDDRLY

SEQ ID NO: 27428 - protein, 9 aa, synthetic construct
GGQGDDRMF

SEQ ID NO: 27429 - protein, 9 aa, synthetic construct
GGGGADYMV

SEQ ID NO: 27430 - protein, 9 aa, synthetic construct
GGEGGDDID

SEQ ID NO: 27431 - protein, 9 aa, synthetic construct
GGQGEDTMF

SEQ ID NO: 27432 - protein, 9 aa, synthetic construct
GGQGEDTLL

SEQ ID NO: 27433 - protein, 9 aa, synthetic construct
GGAGSDTVE

SEQ ID NO: 27434 - protein, 9 aa, synthetic construct
GGGGADVVR

SEQ ID NO: 27435 - protein, 9 aa, synthetic construct
GGAGSDTVL

SEQ ID NO: 27436 - protein, 9 aa, synthetic construct
GGQGEDSFV

SEQ ID NO: 27437 - protein, 9 aa, synthetic construct
GGQGEDQLF

SEQ ID NO: 27438 - protein, 9 aa, synthetic construct
GGQGEDNLY

SEQ ID NO: 27439 - protein, 9 aa, synthetic construct
GGQGEDNLH

SEQ ID NO: 27440 - protein, 9 aa, synthetic construct
GGQGEDMLY

SEQ ID NO: 27441 - protein, 9 aa, synthetic construct
GGQGEDLLT

SEQ ID NO: 27442 - protein, 9 aa, synthetic construct
GGEGGDGLY

SEQ ID NO: 27443 - protein, 9 aa, synthetic construct
GGQGEDKLI

SEQ ID NO: 27444 - protein, 9 aa, synthetic construct
GGQGEDFVQ

SEQ ID NO: 27445 - protein, 9 aa, synthetic construct
GGQGEDFLA

SEQ ID NO: 27446 - protein, 9 aa, synthetic construct
GGAGSDTYT

SEQ ID NO: 27447 - protein, 9 aa, synthetic construct
GGAGSDVAA

SEQ ID NO: 27448 - protein, 9 aa, synthetic construct
GGQGDDYLY

SEQ ID NO: 27449 - protein, 9 aa, synthetic construct
GGEGGDFLD

SEQ ID NO: 27450 - protein, 9 aa, synthetic construct
GGQGEDTVD

SEQ ID NO: 27451 - protein, 9 aa, synthetic construct
GGAGSDTVA

SEQ ID NO: 27452 - protein, 9 aa, synthetic construct
GGQGEDVLD

SEQ ID NO: 27453 - protein, 9 aa, synthetic construct
GGQGFDRLT

SEQ ID NO: 27454 - protein, 9 aa, synthetic construct
GGQGGDLMS

SEQ ID NO: 27455 - protein, 9 aa, synthetic construct
GGQGGDKLG

SEQ ID NO: 27456 - protein, 9 aa, synthetic construct
GGQGGDKLF

SEQ ID NO: 27457 - protein, 9 aa, synthetic construct
GGAGSDTLH

SEQ ID NO: 27458 - protein, 9 aa, synthetic construct
GGQGGDALL

SEQ ID NO: 27459 - protein, 9 aa, synthetic construct
GGQGFDVMD

SEQ ID NO: 27460 - protein, 9 aa, synthetic construct
GGQGFDTLQ

SEQ ID NO: 27461 - protein, 9 aa, synthetic construct
GGQGFDTFV

SEQ ID NO: 27462 - protein, 9 aa, synthetic construct
GGQGFDRLD

SEQ ID NO: 27463 - protein, 9 aa, synthetic construct
GGQGEDVLF

SEQ ID NO: 27464 - protein, 9 aa, synthetic construct
GGQGFDQLY

SEQ ID NO: 27465 - protein, 9 aa, synthetic construct
GGQGFDLLT

SEQ ID NO: 27466 - protein, 9 aa, synthetic construct
GGAGSDTMN

SEQ ID NO: 27467 - protein, 9 aa, synthetic construct
GGQGFDALH

SEQ ID NO: 27468 - protein, 9 aa, synthetic construct
GGAGSDTMQ

SEQ ID NO: 27469 - protein, 9 aa, synthetic construct
GGAGSDTMV

SEQ ID NO: 27470 - protein, 9 aa, synthetic construct
GGQGEDVLY

SEQ ID NO: 27471 - protein, 9 aa, synthetic construct
GGQGEDVLN

SEQ ID NO: 27472 - protein, 9 aa, synthetic construct
GGQGDDYLE

SEQ ID NO: 27473 - protein, 9 aa, synthetic construct
GGQGDDYIS

SEQ ID NO: 27474 - protein, 9 aa, synthetic construct
GGAGSDVAS

SEQ ID NO: 27475 - protein, 9 aa, synthetic construct
GGAGSDVMA

SEQ ID NO: 27476 - protein, 9 aa, synthetic construct
GGQGDDTYD

SEQ ID NO: 27477 - protein, 9 aa, synthetic construct
GGQGDDTVY

SEQ ID NO: 27478 - protein, 9 aa, synthetic construct
GGQGDDTVK

SEQ ID NO: 27479 - protein, 9 aa, synthetic construct
GGQGDDTVG

SEQ ID NO: 27480 - protein, 9 aa, synthetic construct
GGQGDDTVA

SEQ ID NO: 27481 - protein, 9 aa, synthetic construct
GGQGDDTIH

SEQ ID NO: 27482 - protein, 9 aa, synthetic construct
GGQGDDSVT

SEQ ID NO: 27483 - protein, 9 aa, synthetic construct
GGQGDDSVM

SEQ ID NO: 27484 - protein, 9 aa, synthetic construct
GGAGSDVMD

SEQ ID NO: 27485 - protein, 9 aa, synthetic construct
GGAGSDVIT

SEQ ID NO: 27486 - protein, 9 aa, synthetic construct
GGEGGDDML

SEQ ID NO: 27487 - protein, 9 aa, synthetic construct
GGQGDDSLV

SEQ ID NO: 27488 - protein, 9 aa, synthetic construct
GGQGDDSLH

SEQ ID NO: 27489 - protein, 9 aa, synthetic construct
GGAGSDVMK

SEQ ID NO: 27490 - protein, 9 aa, synthetic construct
GGGGADYLN

SEQ ID NO: 27491 - protein, 9 aa, synthetic construct
GGAGSDVMT

SEQ ID NO: 27492 - protein, 9 aa, synthetic construct
GGQGDDSII

SEQ ID NO: 27493 - protein, 9 aa, synthetic construct
GGQGDDSFA

SEQ ID NO: 27494 - protein, 9 aa, synthetic construct
GGQGDDTYG

SEQ ID NO: 27495 - protein, 9 aa, synthetic construct
GGQGDDVFT

SEQ ID NO: 27496 - protein, 9 aa, synthetic construct
GGAGSDVAV

SEQ ID NO: 27497 - protein, 9 aa, synthetic construct
GGQGDDVMV

SEQ ID NO: 27498 - protein, 9 aa, synthetic construct
GGQGDDWLW

SEQ ID NO: 27499 - protein, 9 aa, synthetic construct
GGQGDDWLS

SEQ ID NO: 27500 - protein, 9 aa, synthetic construct
GGQGDDWIE

SEQ ID NO: 27501 - protein, 9 aa, synthetic construct
GGQGDDVYL

SEQ ID NO: 27502 - protein, 9 aa, synthetic construct
GGQGDDVYA

SEQ ID NO: 27503 - protein, 9 aa, synthetic construct
GGGGADYFD

SEQ ID NO: 27504 - protein, 9 aa, synthetic construct
GGQGDDVVV

SEQ ID NO: 27505 - protein, 9 aa, synthetic construct
GGQGDDVVN

SEQ ID NO: 27506 - protein, 9 aa, synthetic construct
GGQGDDVMS

SEQ ID NO: 27507 - protein, 9 aa, synthetic construct
GGGGADYIW

SEQ ID NO: 27508 - protein, 9 aa, synthetic construct
GGEGGDELH

SEQ ID NO: 27509 - protein, 9 aa, synthetic construct
GGQGDDVLG

SEQ ID NO: 27510 - protein, 9 aa, synthetic construct
GGQGDDVLE

SEQ ID NO: 27511 - protein, 9 aa, synthetic construct
GGQGDDVIW

SEQ ID NO: 27512 - protein, 9 aa, synthetic construct
GGQGDDVIT

SEQ ID NO: 27513 - protein, 9 aa, synthetic construct
GGGGADYIS

SEQ ID NO: 27514 - protein, 9 aa, synthetic construct
GGQGDDVIF

SEQ ID NO: 27515 - protein, 9 aa, synthetic construct
GGQGDDVIE

SEQ ID NO: 27516 - protein, 9 aa, synthetic construct
GGQGNDTIF

SEQ ID NO: 27517 - protein, 9 aa, synthetic construct
GGEGADHLD

SEQ ID NO: 27518 - protein, 9 aa, synthetic construct
GGAGSDELR

SEQ ID NO: 27519 - protein, 9 aa, synthetic construct
GGQGRDVLS

SEQ ID NO: 27520 - protein, 9 aa, synthetic construct
GGAGSDELE

SEQ ID NO: 27521 - protein, 9 aa, synthetic construct
GGQGSDLLG

SEQ ID NO: 27522 - protein, 9 aa, synthetic construct
GGQGRDTFV

SEQ ID NO: 27523 - protein, 9 aa, synthetic construct
GGQGRDVLQ

SEQ ID NO: 27524 - protein, 9 aa, synthetic construct
GGGGADSIY

SEQ ID NO: 27525 - protein, 9 aa, synthetic construct
GGAGSDIIH

SEQ ID NO: 27526 - protein, 9 aa, synthetic construct
GGQGNDYLC

SEQ ID NO: 27527 - protein, 9 aa, synthetic construct
GGQGNDVLL

SEQ ID NO: 27528 - protein, 9 aa, synthetic construct
GGQGSDLLE

SEQ ID NO: 27529 - protein, 9 aa, synthetic construct
GGAGSDIIE

SEQ ID NO: 27530 - protein, 9 aa, synthetic construct
GGQGNDVLS

SEQ ID NO: 27531 - protein, 9 aa, synthetic construct
GGAGSDIYR

SEQ ID NO: 27532 - protein, 9 aa, synthetic construct
GGAGSDIID

SEQ ID NO: 27533 - protein, 9 aa, synthetic construct
GGQGQDTFI

SEQ ID NO: 27534 - protein, 9 aa, synthetic construct
GGAGSDEFV

SEQ ID NO: 27535 - protein, 9 aa, synthetic construct
GGGGADTFM

SEQ ID NO: 27536 - protein, 9 aa, synthetic construct
GGAGSDIII

SEQ ID NO: 27537 - protein, 9 aa, synthetic construct
GGAGSDHLI

SEQ ID NO: 27538 - protein, 9 aa, synthetic construct
GGQGNDYLE

SEQ ID NO: 27539 - protein, 9 aa, synthetic construct
GGAGSDKLV

SEQ ID NO: 27540 - protein, 9 aa, synthetic construct
GGQGSDLVD

SEQ ID NO: 27541 - protein, 9 aa, synthetic construct
GGQGNDYLV

SEQ ID NO: 27542 - protein, 9 aa, synthetic construct
GGAGSDFLN

SEQ ID NO: 27543 - protein, 9 aa, synthetic construct
GGQGNDTYR

SEQ ID NO: 27544 - protein, 9 aa, synthetic construct
GGGGADTIK

SEQ ID NO: 27545 - protein, 9 aa, synthetic construct
GGQGRDSIT

SEQ ID NO: 27546 - protein, 9 aa, synthetic construct
GGQGNDYLL

SEQ ID NO: 27547 - protein, 9 aa, synthetic construct
GGQGNDTYT

SEQ ID NO: 27548 - protein, 9 aa, synthetic construct
GGGGADSII

SEQ ID NO: 27549 - protein, 9 aa, synthetic construct
GGQGRDDLL

SEQ ID NO: 27550 - protein, 9 aa, synthetic construct
GGGGADTFY

SEQ ID NO: 27551 - protein, 9 aa, synthetic construct
GGGGADTIM

SEQ ID NO: 27552 - protein, 9 aa, synthetic construct
GGAGSDKLQ

SEQ ID NO: 27553 - protein, 9 aa, synthetic construct
GGQGNDVIS

SEQ ID NO: 27554 - protein, 9 aa, synthetic construct
GGAGSDEIG

SEQ ID NO: 27555 - protein, 9 aa, synthetic construct
GGQGRDVLM

SEQ ID NO: 27556 - protein, 9 aa, synthetic construct
GGQGRDALF

SEQ ID NO: 27557 - protein, 9 aa, synthetic construct
GGQGRDVLK

SEQ ID NO: 27558 - protein, 9 aa, synthetic construct
GGAGSDIAR

SEQ ID NO: 27559 - protein, 9 aa, synthetic construct
GGQGQDVIG

SEQ ID NO: 27560 - protein, 9 aa, synthetic construct
GGQGSDLFI

SEQ ID NO: 27561 - protein, 9 aa, synthetic construct
GGGGADTFS

SEQ ID NO: 27562 - protein, 9 aa, synthetic construct
GGAGSDIAS

SEQ ID NO: 27563 - protein, 9 aa, synthetic construct
GGQGQDVFA

SEQ ID NO: 27564 - protein, 9 aa, synthetic construct
GGQGRDVIS

SEQ ID NO: 27565 - protein, 9 aa, synthetic construct
GGQGQDTLV

SEQ ID NO: 27566 - protein, 9 aa, synthetic construct
GGGGADTIQ

SEQ ID NO: 27567 - protein, 9 aa, synthetic construct
GGAGSDIYY

SEQ ID NO: 27568 - protein, 9 aa, synthetic construct
GGQGRDVLD

SEQ ID NO: 27569 - protein, 9 aa, synthetic construct
GGQGSDKLY

SEQ ID NO: 27570 - protein, 9 aa, synthetic construct
GGQGRDVLE

SEQ ID NO: 27571 - protein, 9 aa, synthetic construct
GGQGSDIYL

SEQ ID NO: 27572 - protein, 9 aa, synthetic construct
GGQGNDWLD

SEQ ID NO: 27573 - protein, 9 aa, synthetic construct
GGAGSDIAG

SEQ ID NO: 27574 - protein, 9 aa, synthetic construct
GGAGSDKAW

SEQ ID NO: 27575 - protein, 9 aa, synthetic construct
GGAGSDIAF

SEQ ID NO: 27576 - protein, 9 aa, synthetic construct
GGQGQDTLE

SEQ ID NO: 27577 - protein, 9 aa, synthetic construct
GGAGSDKLF

SEQ ID NO: 27578 - protein, 9 aa, synthetic construct
GGAGSDIFR

SEQ ID NO: 27579 - protein, 9 aa, synthetic construct
GGQGQDWLE

SEQ ID NO: 27580 - protein, 9 aa, synthetic construct
GGQGQDTLD

SEQ ID NO: 27581 - protein, 9 aa, synthetic construct
GGQGNDVMY

SEQ ID NO: 27582 - protein, 9 aa, synthetic construct
GGQGRDTLS

SEQ ID NO: 27583 - protein, 9 aa, synthetic construct
GGAGSDIYT

SEQ ID NO: 27584 - protein, 9 aa, synthetic construct
GGAGSDIFI

SEQ ID NO: 27585 - protein, 9 aa, synthetic construct
GGQGQDVVF

SEQ ID NO: 27586 - protein, 9 aa, synthetic construct
GGQGSDILH

SEQ ID NO: 27587 - protein, 9 aa, synthetic construct
GGAGSDFIE

SEQ ID NO: 27588 - protein, 9 aa, synthetic construct
GGQGNDWLY

SEQ ID NO: 27589 - protein, 9 aa, synthetic construct
GGGGADSLN

SEQ ID NO: 27590 - protein, 9 aa, synthetic construct
GGAGSDFIA

SEQ ID NO: 27591 - protein, 9 aa, synthetic construct
GGAGSDIVD

SEQ ID NO: 27592 - protein, 9 aa, synthetic construct
GGQGQDRLY

SEQ ID NO: 27593 - protein, 9 aa, synthetic construct
GGAGSDFVD

SEQ ID NO: 27594 - protein, 9 aa, synthetic construct
GGQGPDNMQ

SEQ ID NO: 27595 - protein, 9 aa, synthetic construct
GGGGADSIG

SEQ ID NO: 27596 - protein, 9 aa, synthetic construct
GGAGSDKMM

SEQ ID NO: 27597 - protein, 9 aa, synthetic construct
GGAGSDGID

SEQ ID NO: 27598 - protein, 9 aa, synthetic construct
GGAGSDIMA

SEQ ID NO: 27599 - protein, 9 aa, synthetic construct
GGGGADTLG

SEQ ID NO: 27600 - protein, 9 aa, synthetic construct
GGEGGDRLE

SEQ ID NO: 27601 - protein, 9 aa, synthetic construct
GGQGSDELI

SEQ ID NO: 27602 - protein, 9 aa, synthetic construct
GGQGSDLYL

SEQ ID NO: 27603 - protein, 9 aa, synthetic construct
GGQGNDYVR

SEQ ID NO: 27604 - protein, 9 aa, synthetic construct
GGQGPDAFA

SEQ ID NO: 27605 - protein, 9 aa, synthetic construct
GGQGRDRLE

SEQ ID NO: 27606 - protein, 9 aa, synthetic construct
GGAGSDILE

SEQ ID NO: 27607 - protein, 9 aa, synthetic construct
GGQGNDTVA

SEQ ID NO: 27608 - protein, 9 aa, synthetic construct
GGQGRDLLD

SEQ ID NO: 27609 - protein, 9 aa, synthetic construct
GGQGNDTLG

SEQ ID NO: 27610 - protein, 9 aa, synthetic construct
GGQGNDTMI

SEQ ID NO: 27611 - protein, 9 aa, synthetic construct
GGQGSDHIM

SEQ ID NO: 27612 - protein, 9 aa, synthetic construct
GGAGSDHIS

SEQ ID NO: 27613 - protein, 9 aa, synthetic construct
GGQGQDEIE

SEQ ID NO: 27614 - protein, 9 aa, synthetic construct
GGQGQDLLS

SEQ ID NO: 27615 - protein, 9 aa, synthetic construct
GGQGQDFLA

SEQ ID NO: 27616 - protein, 9 aa, synthetic construct
GGAGSDFAV

SEQ ID NO: 27617 - protein, 9 aa, synthetic construct
GGQGQDFIK

SEQ ID NO: 27618 - protein, 9 aa, synthetic construct
GGGGADTAD

SEQ ID NO: 27619 - protein, 9 aa, synthetic construct
GGAGSDELW

SEQ ID NO: 27620 - protein, 9 aa, synthetic construct
GGQGRDWLK

SEQ ID NO: 27621 - protein, 9 aa, synthetic construct
GGQGPDTFL

SEQ ID NO: 27622 - protein, 9 aa, synthetic construct
GGQGQDRLA

SEQ ID NO: 27623 - protein, 9 aa, synthetic construct
GGGGADSVL

SEQ ID NO: 27624 - protein, 9 aa, synthetic construct
GGQGSDMLD

SEQ ID NO: 27625 - protein, 9 aa, synthetic construct
GGQGRDHLI

SEQ ID NO: 27626 - protein, 9 aa, synthetic construct
GGGGADSVS

SEQ ID NO: 27627 - protein, 9 aa, synthetic construct
GGGGADSVN

SEQ ID NO: 27628 - protein, 9 aa, synthetic construct
GGQGQDQIW

SEQ ID NO: 27629 - protein, 9 aa, synthetic construct
GGQGNDTLH

SEQ ID NO: 27630 - protein, 9 aa, synthetic construct
GGEGGDRLN

SEQ ID NO: 27631 - protein, 9 aa, synthetic construct
GGQGQDLYV

SEQ ID NO: 27632 - protein, 9 aa, synthetic construct
GGAGSDHIL

SEQ ID NO: 27633 - protein, 9 aa, synthetic construct
GGAGSDHFT

SEQ ID NO: 27634 - protein, 9 aa, synthetic construct
GGEGEDELH

SEQ ID NO: 27635 - protein, 9 aa, synthetic construct
GGEGNDHIV

SEQ ID NO: 27636 - protein, 9 aa, synthetic construct
GGEGDDFVS

SEQ ID NO: 27637 - protein, 9 aa, synthetic construct
GGEGDDDLD

SEQ ID NO: 27638 - protein, 9 aa, synthetic construct
GGEGNDSLK

SEQ ID NO: 27639 - protein, 9 aa, synthetic construct
GGEGDDSYI

SEQ ID NO: 27640 - protein, 9 aa, synthetic construct
GGEGNDKII

SEQ ID NO: 27641 - protein, 9 aa, synthetic construct
GGEGIDTAY

SEQ ID NO: 27642 - protein, 9 aa, synthetic construct
GGEGIDSMA

SEQ ID NO: 27643 - protein, 9 aa, synthetic construct
GGEGADWIY

SEQ ID NO: 27644 - protein, 9 aa, synthetic construct
GGEGFDIYA

SEQ ID NO: 27645 - protein, 9 aa, synthetic construct
GGEGDDGLF

SEQ ID NO: 27646 - protein, 9 aa, synthetic construct
GGEGNDYLT

SEQ ID NO: 27647 - protein, 9 aa, synthetic construct
GGEGGDSVD

SEQ ID NO: 27648 - protein, 9 aa, synthetic construct
GGEGDDQLI

SEQ ID NO: 27649 - protein, 9 aa, synthetic construct
GGEGDDSYL

SEQ ID NO: 27650 - protein, 9 aa, synthetic construct
GGEGNDHIT

SEQ ID NO: 27651 - protein, 9 aa, synthetic construct
GGEGEDIVY

SEQ ID NO: 27652 - protein, 9 aa, synthetic construct
GGEGNDHIE

SEQ ID NO: 27653 - protein, 9 aa, synthetic construct
GGEGNDKLM

SEQ ID NO: 27654 - protein, 9 aa, synthetic construct
GGEGFDIAS

SEQ ID NO: 27655 - protein, 9 aa, synthetic construct
GGEGNDYIN

SEQ ID NO: 27656 - protein, 9 aa, synthetic construct
GGEGADKVN

SEQ ID NO: 27657 - protein, 9 aa, synthetic construct
GGEGNDKIF

SEQ ID NO: 27658 - protein, 9 aa, synthetic construct
GGEGIDTFN

SEQ ID NO: 27659 - protein, 9 aa, synthetic construct
GGEGHDTAD

SEQ ID NO: 27660 - protein, 9 aa, synthetic construct
GGEGDDQLK

SEQ ID NO: 27661 - protein, 9 aa, synthetic construct
GGEGNDKFV

SEQ ID NO: 27662 - protein, 9 aa, synthetic construct
GGEGADIVQ

SEQ ID NO: 27663 - protein, 9 aa, synthetic construct
GGEGNDYIF

SEQ ID NO: 27664 - protein, 9 aa, synthetic construct
GGEGFDKLD

SEQ ID NO: 27665 - protein, 9 aa, synthetic construct
GGEGADWLD

SEQ ID NO: 27666 - protein, 9 aa, synthetic construct
GGEGHDTAL

SEQ ID NO: 27667 - protein, 9 aa, synthetic construct
GGEGDDDLA

SEQ ID NO: 27668 - protein, 9 aa, synthetic construct
GGEGGDDIL

SEQ ID NO: 27669 - protein, 9 aa, synthetic construct
GGEGMDLFA

SEQ ID NO: 27670 - protein, 9 aa, synthetic construct
GGEGDDSVE

SEQ ID NO: 27671 - protein, 9 aa, synthetic construct
GGEGADIVV

SEQ ID NO: 27672 - protein, 9 aa, synthetic construct
GGEGGDDLA

SEQ ID NO: 27673 - protein, 9 aa, synthetic construct
GGEGNDHLA

SEQ ID NO: 27674 - protein, 9 aa, synthetic construct
GGEGNDYLH

SEQ ID NO: 27675 - protein, 9 aa, synthetic construct
GGEGEDIVE

SEQ ID NO: 27676 - protein, 9 aa, synthetic construct
GGEGEDELF

SEQ ID NO: 27677 - protein, 9 aa, synthetic construct
GGEGADKIW

SEQ ID NO: 27678 - protein, 9 aa, synthetic construct
GGEGADKIV

SEQ ID NO: 27679 - protein, 9 aa, synthetic construct
GGEGGDDLL

SEQ ID NO: 27680 - protein, 9 aa, synthetic construct
GGEGDDSVD

SEQ ID NO: 27681 - protein, 9 aa, synthetic construct
GGEGNDKLD

SEQ ID NO: 27682 - protein, 9 aa, synthetic construct
GGEGADKIG

SEQ ID NO: 27683 - protein, 9 aa, synthetic construct
GGEGADKID

SEQ ID NO: 27684 - protein, 9 aa, synthetic construct
GGEGIDTAA

SEQ ID NO: 27685 - protein, 9 aa, synthetic construct
GGEGDDQFV

SEQ ID NO: 27686 - protein, 9 aa, synthetic construct
GGEGFDIVS

SEQ ID NO: 27687 - protein, 9 aa, synthetic construct
GGEGIDTAG

SEQ ID NO: 27688 - protein, 9 aa, synthetic construct
GGEGEDILY

SEQ ID NO: 27689 - protein, 9 aa, synthetic construct
GGEGADIYV

SEQ ID NO: 27690 - protein, 9 aa, synthetic construct
GGEGNDYLK

SEQ ID NO: 27691 - protein, 9 aa, synthetic construct
GGEGNDSLQ

SEQ ID NO: 27692 - protein, 9 aa, synthetic construct
GGEGHDTIY

SEQ ID NO: 27693 - protein, 9 aa, synthetic construct
GGEGADKFQ

SEQ ID NO: 27694 - protein, 9 aa, synthetic construct
GGEGDDCVS

SEQ ID NO: 27695 - protein, 9 aa, synthetic construct
GGEGDDSMT

SEQ ID NO: 27696 - protein, 9 aa, synthetic construct
GGEGDDSVW

SEQ ID NO: 27697 - protein, 9 aa, synthetic construct
GGEGADKLF

SEQ ID NO: 27698 - protein, 9 aa, synthetic construct
GGEGIDTAV

SEQ ID NO: 27699 - protein, 9 aa, synthetic construct
GGEGDDEVL

SEQ ID NO: 27700 - protein, 9 aa, synthetic construct
GGEGIDTAR

SEQ ID NO: 27701 - protein, 9 aa, synthetic construct
GGEGFDILT

SEQ ID NO: 27702 - protein, 9 aa, synthetic construct
GGEGEDELN

SEQ ID NO: 27703 - protein, 9 aa, synthetic construct
GGEGHDTFR

SEQ ID NO: 27704 - protein, 9 aa, synthetic construct
GGEGFDILV

SEQ ID NO: 27705 - protein, 9 aa, synthetic construct
GGEGDDQIR

SEQ ID NO: 27706 - protein, 9 aa, synthetic construct
GGEGIDTAM

SEQ ID NO: 27707 - protein, 9 aa, synthetic construct
GGEGDDSVN

SEQ ID NO: 27708 - protein, 9 aa, synthetic construct
GGEGNDYIW

SEQ ID NO: 27709 - protein, 9 aa, synthetic construct
GGEGDDEMT

SEQ ID NO: 27710 - protein, 9 aa, synthetic construct
GGEGADIVS

SEQ ID NO: 27711 - protein, 9 aa, synthetic construct
GGEGHDTLH

SEQ ID NO: 27712 - protein, 9 aa, synthetic construct
GGEGMDIFI

SEQ ID NO: 27713 - protein, 9 aa, synthetic construct
GGEGGDRLM

SEQ ID NO: 27714 - protein, 9 aa, synthetic construct
GGEGDDQFI

SEQ ID NO: 27715 - protein, 9 aa, synthetic construct
GGEGHDTIQ

SEQ ID NO: 27716 - protein, 9 aa, synthetic construct
GGEGNDKLG

SEQ ID NO: 27717 - protein, 9 aa, synthetic construct
GGEGNDKIT

SEQ ID NO: 27718 - protein, 9 aa, synthetic construct
GGEGADKLS

SEQ ID NO: 27719 - protein, 9 aa, synthetic construct
GGEGADKLR

SEQ ID NO: 27720 - protein, 9 aa, synthetic construct
GGEGFDIVL

SEQ ID NO: 27721 - protein, 9 aa, synthetic construct
GGEGNDKLN

SEQ ID NO: 27722 - protein, 9 aa, synthetic construct
GGEGIDTID

SEQ ID NO: 27723 - protein, 9 aa, synthetic construct
GGEGFDGLY

SEQ ID NO: 27724 - protein, 9 aa, synthetic construct
GGEGHDRLS

SEQ ID NO: 27725 - protein, 9 aa, synthetic construct
GGEGDDHLH

SEQ ID NO: 27726 - protein, 9 aa, synthetic construct
GGEGDDAVW

SEQ ID NO: 27727 - protein, 9 aa, synthetic construct
GGEGGDSVL

SEQ ID NO: 27728 - protein, 9 aa, synthetic construct
GGEGDDNLR

SEQ ID NO: 27729 - protein, 9 aa, synthetic construct
GGEGDDNLQ

SEQ ID NO: 27730 - protein, 9 aa, synthetic construct
GGEGNDRMS

SEQ ID NO: 27731 - protein, 9 aa, synthetic construct
GGEGGDHLS

SEQ ID NO: 27732 - protein, 9 aa, synthetic construct
GGEGNDFVF

SEQ ID NO: 27733 - protein, 9 aa, synthetic construct
GGEGHDRLI

SEQ ID NO: 27734 - protein, 9 aa, synthetic construct
GGEGNDFLV

SEQ ID NO: 27735 - protein, 9 aa, synthetic construct
GGEGDDNLL

SEQ ID NO: 27736 - protein, 9 aa, synthetic construct
GGEGDDNLK

SEQ ID NO: 27737 - protein, 9 aa, synthetic construct
GGEGNDAIV

SEQ ID NO: 27738 - protein, 9 aa, synthetic construct
GGEGDDAVR

SEQ ID NO: 27739 - protein, 9 aa, synthetic construct
GGEGNDVYV

SEQ ID NO: 27740 - protein, 9 aa, synthetic construct
GGEGNDKVF

SEQ ID NO: 27741 - protein, 9 aa, synthetic construct
GGEGGDDVD

SEQ ID NO: 27742 - protein, 9 aa, synthetic construct
GGEGNDKVD

SEQ ID NO: 27743 - protein, 9 aa, synthetic construct
GGEGNDSMY

SEQ ID NO: 27744 - protein, 9 aa, synthetic construct
GGEGDDNLW

SEQ ID NO: 27745 - protein, 9 aa, synthetic construct
GGEGHDSIR

SEQ ID NO: 27746 - protein, 9 aa, synthetic construct
GGEGIDTVR

SEQ ID NO: 27747 - protein, 9 aa, synthetic construct
GGEGDDKIE

SEQ ID NO: 27748 - protein, 9 aa, synthetic construct
GGEGNDWAA

SEQ ID NO: 27749 - protein, 9 aa, synthetic construct
GGEGCDLLE

SEQ ID NO: 27750 - protein, 9 aa, synthetic construct
GGEGDDELQ

SEQ ID NO: 27751 - protein, 9 aa, synthetic construct
GGEGDDTIQ

SEQ ID NO: 27752 - protein, 9 aa, synthetic construct
GGEGIDVLI

SEQ ID NO: 27753 - protein, 9 aa, synthetic construct
GGEGIDVLL

SEQ ID NO: 27754 - protein, 9 aa, synthetic construct
GGEGHDSFG

SEQ ID NO: 27755 - protein, 9 aa, synthetic construct
GGEGEDKLI

SEQ ID NO: 27756 - protein, 9 aa, synthetic construct
GGEGHDRVS

SEQ ID NO: 27757 - protein, 9 aa, synthetic construct
GGEGCDQFV

SEQ ID NO: 27758 - protein, 9 aa, synthetic construct
GGEGDDDLI

SEQ ID NO: 27759 - protein, 9 aa, synthetic construct
GGEGADLIT

SEQ ID NO: 27760 - protein, 9 aa, synthetic construct
GGEGHDRAS

SEQ ID NO: 27761 - protein, 9 aa, synthetic construct
GGEGADWIF

SEQ ID NO: 27762 - protein, 9 aa, synthetic construct
GGEGHDRFM

SEQ ID NO: 27763 - protein, 9 aa, synthetic construct
GGEGFDFLF

SEQ ID NO: 27764 - protein, 9 aa, synthetic construct
GGEGIDWAS

SEQ ID NO: 27765 - protein, 9 aa, synthetic construct
GGEGIDWLD

SEQ ID NO: 27766 - protein, 9 aa, synthetic construct
GGEGEDALH

SEQ ID NO: 27767 - protein, 9 aa, synthetic construct
GGEGNDLFH

SEQ ID NO: 27768 - protein, 9 aa, synthetic construct
GGEGGDHLY

SEQ ID NO: 27769 - protein, 9 aa, synthetic construct
GGEGDDNIT

SEQ ID NO: 27770 - protein, 9 aa, synthetic construct
GGEGFDFAW

SEQ ID NO: 27771 - protein, 9 aa, synthetic construct
GGEGNDSYS

SEQ ID NO: 27772 - protein, 9 aa, synthetic construct
GGEGHDQML

SEQ ID NO: 27773 - protein, 9 aa, synthetic construct
GGEGIDWLY

SEQ ID NO: 27774 - protein, 9 aa, synthetic construct
GGEGDDDLL

SEQ ID NO: 27775 - protein, 9 aa, synthetic construct
GGEGNDLFF

SEQ ID NO: 27776 - protein, 9 aa, synthetic construct
GGEGHDRIL

SEQ ID NO: 27777 - protein, 9 aa, synthetic construct
GGEGDDNLE

SEQ ID NO: 27778 - protein, 9 aa, synthetic construct
GGEGDDAVE

SEQ ID NO: 27779 - protein, 9 aa, synthetic construct
GGEGHDRLF

SEQ ID NO: 27780 - protein, 9 aa, synthetic construct
GGEGNDFLQ

SEQ ID NO: 27781 - protein, 9 aa, synthetic construct
GGEGLDVIA

SEQ ID NO: 27782 - protein, 9 aa, synthetic construct
GGEGIDVVF

SEQ ID NO: 27783 - protein, 9 aa, synthetic construct
GGEGCDSLT

SEQ ID NO: 27784 - protein, 9 aa, synthetic construct
GGEGLDVLR

SEQ ID NO: 27785 - protein, 9 aa, synthetic construct
GGEGCDQLD

SEQ ID NO: 27786 - protein, 9 aa, synthetic construct
GGEGNDRMR

SEQ ID NO: 27787 - protein, 9 aa, synthetic construct
GGEGLDVLW

SEQ ID NO: 27788 - protein, 9 aa, synthetic construct
GGEGEDLIE

SEQ ID NO: 27789 - protein, 9 aa, synthetic construct
GGEGNDLAR

SEQ ID NO: 27790 - protein, 9 aa, synthetic construct
GGEGGDHME

SEQ ID NO: 27791 - protein, 9 aa, synthetic construct
GGEGGDTAD

SEQ ID NO: 27792 - protein, 9 aa, synthetic construct
GGEGHDSIY

SEQ ID NO: 27793 - protein, 9 aa, synthetic construct
GGEGNDWIF

SEQ ID NO: 27794 - protein, 9 aa, synthetic construct
GGEGEDALL

SEQ ID NO: 27795 - protein, 9 aa, synthetic construct
GGEGNDGLN

SEQ ID NO: 27796 - protein, 9 aa, synthetic construct
GGEGMDLFS

SEQ ID NO: 27797 - protein, 9 aa, synthetic construct
GGEGDDGMT

SEQ ID NO: 27798 - protein, 9 aa, synthetic construct
GGEGDDPIK

SEQ ID NO: 27799 - protein, 9 aa, synthetic construct
GGEGDDNVQ

SEQ ID NO: 27800 - protein, 9 aa, synthetic construct
GGEGDDTAV

SEQ ID NO: 27801 - protein, 9 aa, synthetic construct
GGEGDDTFD

SEQ ID NO: 27802 - protein, 9 aa, synthetic construct
GGEGEDEIL

SEQ ID NO: 27803 - protein, 9 aa, synthetic construct
GGEGNDSMD

SEQ ID NO: 27804 - protein, 9 aa, synthetic construct
GGEGGDDVT

SEQ ID NO: 27805 - protein, 9 aa, synthetic construct
GGEGHDSMA

SEQ ID NO: 27806 - protein, 9 aa, synthetic construct
GGEGNDSMA

SEQ ID NO: 27807 - protein, 9 aa, synthetic construct
GGEGNDWLW

SEQ ID NO: 27808 - protein, 9 aa, synthetic construct
GGEGNDWLV

SEQ ID NO: 27809 - protein, 9 aa, synthetic construct
GGEGDDTFE

SEQ ID NO: 27810 - protein, 9 aa, synthetic construct
GGEGIDTIA

SEQ ID NO: 27811 - protein, 9 aa, synthetic construct
GGEGDDGMP

SEQ ID NO: 27812 - protein, 9 aa, synthetic construct
GGEGNDKLQ

SEQ ID NO: 27813 - protein, 9 aa, synthetic construct
GGEGADWIS

SEQ ID NO: 27814 - protein, 9 aa, synthetic construct
GGEGDDGLY

SEQ ID NO: 27815 - protein, 9 aa, synthetic construct
GGEGDDTAK

SEQ ID NO: 27816 - protein, 9 aa, synthetic construct
GGEGDDTAI

SEQ ID NO: 27817 - protein, 9 aa, synthetic construct
GGEGNDWVL

SEQ ID NO: 27818 - protein, 9 aa, synthetic construct
GGEGDDGLR

SEQ ID NO: 27819 - protein, 9 aa, synthetic construct
GGEGNDYAF

SEQ ID NO: 27820 - protein, 9 aa, synthetic construct
GGEGDDQAL

SEQ ID NO: 27821 - protein, 9 aa, synthetic construct
GGEGNDYFN

SEQ ID NO: 27822 - protein, 9 aa, synthetic construct
GGEGDDGLL

SEQ ID NO: 27823 - protein, 9 aa, synthetic construct
GGEGIDTFV

SEQ ID NO: 27824 - protein, 9 aa, synthetic construct
GGEGDDKFT

SEQ ID NO: 27825 - protein, 9 aa, synthetic construct
GGEGNDYFW

SEQ ID NO: 27826 - protein, 9 aa, synthetic construct
GGEGDDGLG

SEQ ID NO: 27827 - protein, 9 aa, synthetic construct
GGEGFDFLN

SEQ ID NO: 27828 - protein, 9 aa, synthetic construct
GGEGGDRLL

SEQ ID NO: 27829 - protein, 9 aa, synthetic construct
GGEGIDTMV

SEQ ID NO: 27830 - protein, 9 aa, synthetic construct
GGEGFDFLL

SEQ ID NO: 27831 - protein, 9 aa, synthetic construct
GGEGIDTMI

SEQ ID NO: 27832 - protein, 9 aa, synthetic construct
GGEGEDDLD

SEQ ID NO: 27833 - protein, 9 aa, synthetic construct
GGEGGDRLI

SEQ ID NO: 27834 - protein, 9 aa, synthetic construct
GGEGDDTFS

SEQ ID NO: 27835 - protein, 9 aa, synthetic construct
GGEGDDCLV

SEQ ID NO: 27836 - protein, 9 aa, synthetic construct
GGEGIDTMT

SEQ ID NO: 27837 - protein, 9 aa, synthetic construct
GGEGDDCLT

SEQ ID NO: 27838 - protein, 9 aa, synthetic construct
GGEGHDSLW

SEQ ID NO: 27839 - protein, 9 aa, synthetic construct
GGEGNDSMT

SEQ ID NO: 27840 - protein, 9 aa, synthetic construct
GGEGDDKFY

SEQ ID NO: 27841 - protein, 9 aa, synthetic construct
GGEGHDSLF

SEQ ID NO: 27842 - protein, 9 aa, synthetic construct
GGEGNDWIS

SEQ ID NO: 27843 - protein, 9 aa, synthetic construct
GGEGHDSLD

SEQ ID NO: 27844 - protein, 9 aa, synthetic construct
GGEGNDWIQ

SEQ ID NO: 27845 - protein, 9 aa, synthetic construct
GGEGNDSML

SEQ ID NO: 27846 - protein, 9 aa, synthetic construct
GGEGADRMD

SEQ ID NO: 27847 - protein, 9 aa, synthetic construct
GGEGDDHIV

SEQ ID NO: 27848 - protein, 9 aa, synthetic construct
GGEGEDDMT

SEQ ID NO: 27849 - protein, 9 aa, synthetic construct
GGEGDDTFH

SEQ ID NO: 27850 - protein, 9 aa, synthetic construct
GGEGADRMN

SEQ ID NO: 27851 - protein, 9 aa, synthetic construct
GGEGDDHIH

SEQ ID NO: 27852 - protein, 9 aa, synthetic construct
GGEGIDTLV

SEQ ID NO: 27853 - protein, 9 aa, synthetic construct
GGEGDDHIE

SEQ ID NO: 27854 - protein, 9 aa, synthetic construct
GGEGNDSMI

SEQ ID NO: 27855 - protein, 9 aa, synthetic construct
GGEGGDFAQ

SEQ ID NO: 27856 - protein, 9 aa, synthetic construct
GGEGADRMT

SEQ ID NO: 27857 - protein, 9 aa, synthetic construct
GGEGNDGIY

SEQ ID NO: 27858 - protein, 9 aa, synthetic construct
GGEGDDHFT

SEQ ID NO: 27859 - protein, 9 aa, synthetic construct
GGEGIDTLI

SEQ ID NO: 27860 - protein, 9 aa, synthetic construct
GGEGIDTLE

SEQ ID NO: 27861 - protein, 9 aa, synthetic construct
GGEGHDSLV

SEQ ID NO: 27862 - protein, 9 aa, synthetic construct
GGEGNDYMD

SEQ ID NO: 27863 - protein, 9 aa, synthetic construct
GGEGNDTFT

SEQ ID NO: 27864 - protein, 9 aa, synthetic construct
GGEGGDALD

SEQ ID NO: 27865 - protein, 9 aa, synthetic construct
GGEGQDILA

SEQ ID NO: 27866 - protein, 9 aa, synthetic construct
GGEGNDSII

SEQ ID NO: 27867 - protein, 9 aa, synthetic construct
GGEGFDVVS

SEQ ID NO: 27868 - protein, 9 aa, synthetic construct
GGEGHDYVY

SEQ ID NO: 27869 - protein, 9 aa, synthetic construct
GGEGFDTAI

SEQ ID NO: 27870 - protein, 9 aa, synthetic construct
GGEGIDLAS

SEQ ID NO: 27871 - protein, 9 aa, synthetic construct
GGEGHDYMN

SEQ ID NO: 27872 - protein, 9 aa, synthetic construct
GGEGQDILS

SEQ ID NO: 27873 - protein, 9 aa, synthetic construct
GGEGIDLLD

SEQ ID NO: 27874 - protein, 9 aa, synthetic construct
GGEGIDLLF

SEQ ID NO: 27875 - protein, 9 aa, synthetic construct
GGEGFDTAA

SEQ ID NO: 27876 - protein, 9 aa, synthetic construct
GGEGDDRIH

SEQ ID NO: 27877 - protein, 9 aa, synthetic construct
GGEGQDILL

SEQ ID NO: 27878 - protein, 9 aa, synthetic construct
GGEGGDRYV

SEQ ID NO: 27879 - protein, 9 aa, synthetic construct
GGEGIDLLV

SEQ ID NO: 27880 - protein, 9 aa, synthetic construct
GGEGADTLW

SEQ ID NO: 27881 - protein, 9 aa, synthetic construct
GGEGIDALY

SEQ ID NO: 27882 - protein, 9 aa, synthetic construct
GGEGFDVLS

SEQ ID NO: 27883 - protein, 9 aa, synthetic construct
GGEGADYIK

SEQ ID NO: 27884 - protein, 9 aa, synthetic construct
GGEGDDRIR

SEQ ID NO: 27885 - protein, 9 aa, synthetic construct
GGEGDDSIA

SEQ ID NO: 27886 - protein, 9 aa, synthetic construct
GGEGFDVAD

SEQ ID NO: 27887 - protein, 9 aa, synthetic construct
GGEGIDFAS

SEQ ID NO: 27888 - protein, 9 aa, synthetic construct
GGEGEDGLF

SEQ ID NO: 27889 - protein, 9 aa, synthetic construct
GGEGIDELI

SEQ ID NO: 27890 - protein, 9 aa, synthetic construct
GGEGDDSIH

SEQ ID NO: 27891 - protein, 9 aa, synthetic construct
GGEGEDIFV

SEQ ID NO: 27892 - protein, 9 aa, synthetic construct
GGEGADIAV

SEQ ID NO: 27893 - protein, 9 aa, synthetic construct
GGEGQDLFL

SEQ ID NO: 27894 - protein, 9 aa, synthetic construct
GGEGNDRVE

SEQ ID NO: 27895 - protein, 9 aa, synthetic construct
GGEGIDDLQ

SEQ ID NO: 27896 - protein, 9 aa, synthetic construct
GGEGADYIN

SEQ ID NO: 27897 - protein, 9 aa, synthetic construct
GGEGGDRMD

SEQ ID NO: 27898 - protein, 9 aa, synthetic construct
GGEGDDRIK

SEQ ID NO: 27899 - protein, 9 aa, synthetic construct
GGEGFDSYE

SEQ ID NO: 27900 - protein, 9 aa, synthetic construct
GGEGMDVFI

SEQ ID NO: 27901 - protein, 9 aa, synthetic construct
GGEGADSII

SEQ ID NO: 27902 - protein, 9 aa, synthetic construct
GGEGQDIAK

SEQ ID NO: 27903 - protein, 9 aa, synthetic construct
GGEGQDELR

SEQ ID NO: 27904 - protein, 9 aa, synthetic construct
GGEGQDELL

SEQ ID NO: 27905 - protein, 9 aa, synthetic construct
GGEGFDRLF

SEQ ID NO: 27906 - protein, 9 aa, synthetic construct
GGEGMDTLY

SEQ ID NO: 27907 - protein, 9 aa, synthetic construct
GGEGQDEAT

SEQ ID NO: 27908 - protein, 9 aa, synthetic construct
GGEGADSFI

SEQ ID NO: 27909 - protein, 9 aa, synthetic construct
GGEGADSFF

SEQ ID NO: 27910 - protein, 9 aa, synthetic construct
GGEGQDDLW

SEQ ID NO: 27911 - protein, 9 aa, synthetic construct
GGEGNDHVH

SEQ ID NO: 27912 - protein, 9 aa, synthetic construct
GGEGMDTLN

SEQ ID NO: 27913 - protein, 9 aa, synthetic construct
GGEGADTVA

SEQ ID NO: 27914 - protein, 9 aa, synthetic construct
GGEGMDTLL

SEQ ID NO: 27915 - protein, 9 aa, synthetic construct
GGEGMDTLF

SEQ ID NO: 27916 - protein, 9 aa, synthetic construct
GGEGNDSIQ

SEQ ID NO: 27917 - protein, 9 aa, synthetic construct
GGEGDDSLM

SEQ ID NO: 27918 - protein, 9 aa, synthetic construct
GGEGADSFQ

SEQ ID NO: 27919 - protein, 9 aa, synthetic construct
GGEGADSFS

SEQ ID NO: 27920 - protein, 9 aa, synthetic construct
GGEGQDFAS

SEQ ID NO: 27921 - protein, 9 aa, synthetic construct
GGEGADYIE

SEQ ID NO: 27922 - protein, 9 aa, synthetic construct
GGEGFDSVT

SEQ ID NO: 27923 - protein, 9 aa, synthetic construct
GGEGNDIAE

SEQ ID NO: 27924 - protein, 9 aa, synthetic construct
GGEGNDRVD

SEQ ID NO: 27925 - protein, 9 aa, synthetic construct
GGEGNDHYV

SEQ ID NO: 27926 - protein, 9 aa, synthetic construct
GGEGIDLME

SEQ ID NO: 27927 - protein, 9 aa, synthetic construct
GGEGFDRMY

SEQ ID NO: 27928 - protein, 9 aa, synthetic construct
GGEGHDWLS

SEQ ID NO: 27929 - protein, 9 aa, synthetic construct
GGEGQDFIY

SEQ ID NO: 27930 - protein, 9 aa, synthetic construct
GGEGFDRLS

SEQ ID NO: 27931 - protein, 9 aa, synthetic construct
GGEGNDHYI

SEQ ID NO: 27932 - protein, 9 aa, synthetic construct
GGEGDDFLG

SEQ ID NO: 27933 - protein, 9 aa, synthetic construct
GGEGDDFLH

SEQ ID NO: 27934 - protein, 9 aa, synthetic construct
GGEGQDGYM

SEQ ID NO: 27935 - protein, 9 aa, synthetic construct
GGEGQDFLF

SEQ ID NO: 27936 - protein, 9 aa, synthetic construct
GGEGNDILC

SEQ ID NO: 27937 - protein, 9 aa, synthetic construct
GGEGIDKLR

SEQ ID NO: 27938 - protein, 9 aa, synthetic construct
GGEGDDSMR

SEQ ID NO: 27939 - protein, 9 aa, synthetic construct
GGEGQDNLR

SEQ ID NO: 27940 - protein, 9 aa, synthetic construct
GGEGFDTLN

SEQ ID NO: 27941 - protein, 9 aa, synthetic construct
GGEGNDIFI

SEQ ID NO: 27942 - protein, 9 aa, synthetic construct
GGEGDDDIT

SEQ ID NO: 27943 - protein, 9 aa, synthetic construct
GGEGDDFIS

SEQ ID NO: 27944 - protein, 9 aa, synthetic construct
GGEGFDTIA

SEQ ID NO: 27945 - protein, 9 aa, synthetic construct
GGEGNDRVM

SEQ ID NO: 27946 - protein, 9 aa, synthetic construct
GGEGDDFIA

SEQ ID NO: 27947 - protein, 9 aa, synthetic construct
GGEGFDTLQ

SEQ ID NO: 27948 - protein, 9 aa, synthetic construct
GGEGNDRVI

SEQ ID NO: 27949 - protein, 9 aa, synthetic construct
GGEGNDSAY

SEQ ID NO: 27950 - protein, 9 aa, synthetic construct
GGEGQDQLE

SEQ ID NO: 27951 - protein, 9 aa, synthetic construct
GGEGNDIIN

SEQ ID NO: 27952 - protein, 9 aa, synthetic construct
GGEGNDIIQ

SEQ ID NO: 27953 - protein, 9 aa, synthetic construct
GGEGEDHLV

SEQ ID NO: 27954 - protein, 9 aa, synthetic construct
GGEGQDQIF

SEQ ID NO: 27955 - protein, 9 aa, synthetic construct
GGEGDDDIV

SEQ ID NO: 27956 - protein, 9 aa, synthetic construct
GGEGNDIIH

SEQ ID NO: 27957 - protein, 9 aa, synthetic construct
GGEGNDRVY

SEQ ID NO: 27958 - protein, 9 aa, synthetic construct
GGEGFDTID

SEQ ID NO: 27959 - protein, 9 aa, synthetic construct
GGEGQDRLL

SEQ ID NO: 27960 - protein, 9 aa, synthetic construct
GGEGIDILY

SEQ ID NO: 27961 - protein, 9 aa, synthetic construct
GGEGNDIFS

SEQ ID NO: 27962 - protein, 9 aa, synthetic construct
GGEGFDTLI

SEQ ID NO: 27963 - protein, 9 aa, synthetic construct
GGEGQDRLD

SEQ ID NO: 27964 - protein, 9 aa, synthetic construct
GGEGQDRIY

SEQ ID NO: 27965 - protein, 9 aa, synthetic construct
GGEGADSIW

SEQ ID NO: 27966 - protein, 9 aa, synthetic construct
GGEGADHLK

SEQ ID NO: 27967 - protein, 9 aa, synthetic construct
GGEGADHLF

SEQ ID NO: 27968 - protein, 9 aa, synthetic construct
GGEGNDRYY

SEQ ID NO: 27969 - protein, 9 aa, synthetic construct
GGEGADTMS

SEQ ID NO: 27970 - protein, 9 aa, synthetic construct
GGEGQDRFM

SEQ ID NO: 27971 - protein, 9 aa, synthetic construct
GGEGQDRFE

SEQ ID NO: 27972 - protein, 9 aa, synthetic construct
GGEGDDFII

SEQ ID NO: 27973 - protein, 9 aa, synthetic construct
GGEGDDFFS

SEQ ID NO: 27974 - protein, 9 aa, synthetic construct
GGEGDDFFH

SEQ ID NO: 27975 - protein, 9 aa, synthetic construct
GGEGFDTYY

SEQ ID NO: 27976 - protein, 9 aa, synthetic construct
GGEGEDHLL

SEQ ID NO: 27977 - protein, 9 aa, synthetic construct
GGEGDDDIN

SEQ ID NO: 27978 - protein, 9 aa, synthetic construct
GGEGIDILI

SEQ ID NO: 27979 - protein, 9 aa, synthetic construct
GGEGDDRYY

SEQ ID NO: 27980 - protein, 9 aa, synthetic construct
GGEGIDILD

SEQ ID NO: 27981 - protein, 9 aa, synthetic construct
GGEGDDSAA

SEQ ID NO: 27982 - protein, 9 aa, synthetic construct
GGEGDDSAD

SEQ ID NO: 27983 - protein, 9 aa, synthetic construct
GGEGDDSFF

SEQ ID NO: 27984 - protein, 9 aa, synthetic construct
GGEGGDRLT

SEQ ID NO: 27985 - protein, 9 aa, synthetic construct
GGEGQDLLH

SEQ ID NO: 27986 - protein, 9 aa, synthetic construct
GGEGIDIAS

SEQ ID NO: 27987 - protein, 9 aa, synthetic construct
GGEGADYLE

SEQ ID NO: 27988 - protein, 9 aa, synthetic construct
GGEGDDRIV

SEQ ID NO: 27989 - protein, 9 aa, synthetic construct
GGEGQDLLE

SEQ ID NO: 27990 - protein, 9 aa, synthetic construct
GGEGDDSFT

SEQ ID NO: 27991 - protein, 9 aa, synthetic construct
GGEGDDSFY

SEQ ID NO: 27992 - protein, 9 aa, synthetic construct
GGEGDDFLE

SEQ ID NO: 27993 - protein, 9 aa, synthetic construct
GGEGFDTYT

SEQ ID NO: 27994 - protein, 9 aa, synthetic construct
GGEGDDRVY

SEQ ID NO: 27995 - protein, 9 aa, synthetic construct
GGEGQDLVD

SEQ ID NO: 27996 - protein, 9 aa, synthetic construct
GGEGEDHLD

SEQ ID NO: 27997 - protein, 9 aa, synthetic construct
GGEGGDRLQ

SEQ ID NO: 27998 - protein, 9 aa, synthetic construct
GGEGFDTFY

SEQ ID NO: 27999 - protein, 9 aa, synthetic construct
GGEGDDRMT

SEQ ID NO: 28000 - protein, 9 aa, synthetic construct
GGEGQDMLL

SEQ ID NO: 28001 - protein, 9 aa, synthetic construct
GGEGMDWLV

SEQ ID NO: 28002 - protein, 9 aa, synthetic construct
GGEGADHMY

SEQ ID NO: 28003 - protein, 9 aa, synthetic construct
GGEGDDRVV

SEQ ID NO: 28004 - protein, 9 aa, synthetic construct
GGEGADYLL

SEQ ID NO: 28005 - protein, 9 aa, synthetic construct
GGEGNDSFY

SEQ ID NO: 28006 - protein, 9 aa, synthetic construct
GGEGDDRVS

SEQ ID NO: 28007 - protein, 9 aa, synthetic construct
GGEGDDDIS

SEQ ID NO: 28008 - protein, 9 aa, synthetic construct
GGEGNDRVH

SEQ ID NO: 28009 - protein, 9 aa, synthetic construct
GGEGNDSIA

SEQ ID NO: 28010 - protein, 9 aa, synthetic construct
GGEGMDTLD

SEQ ID NO: 28011 - protein, 9 aa, synthetic construct
GGEGHDWLF

SEQ ID NO: 28012 - protein, 9 aa, synthetic construct
GGEGQDALR

SEQ ID NO: 28013 - protein, 9 aa, synthetic construct
GGEGEDFID

SEQ ID NO: 28014 - protein, 9 aa, synthetic construct
GGEGMDMLI

SEQ ID NO: 28015 - protein, 9 aa, synthetic construct
GGEGHDVLA

SEQ ID NO: 28016 - protein, 9 aa, synthetic construct
GGEGPDLIF

SEQ ID NO: 28017 - protein, 9 aa, synthetic construct
GGEGHDVIY

SEQ ID NO: 28018 - protein, 9 aa, synthetic construct
GGEGNDSIW

SEQ ID NO: 28019 - protein, 9 aa, synthetic construct
GGEGHDVIH

SEQ ID NO: 28020 - protein, 9 aa, synthetic construct
GGEGDDFVA

SEQ ID NO: 28021 - protein, 9 aa, synthetic construct
GGEGHDVAL

SEQ ID NO: 28022 - protein, 9 aa, synthetic construct
GGEGDDSMD

SEQ ID NO: 28023 - protein, 9 aa, synthetic construct
GGEGHDTVD

SEQ ID NO: 28024 - protein, 9 aa, synthetic construct
GGEGHDTVA

SEQ ID NO: 28025 - protein, 9 aa, synthetic construct
GGEGDDSMI

SEQ ID NO: 28026 - protein, 9 aa, synthetic construct
GGEGDDFVD

SEQ ID NO: 28027 - protein, 9 aa, synthetic construct
GGEGIDRFV

SEQ ID NO: 28028 - protein, 9 aa, synthetic construct
GGEGEDIIL

SEQ ID NO: 28029 - protein, 9 aa, synthetic construct
GGEGADRYL

SEQ ID NO: 28030 - protein, 9 aa, synthetic construct
GGEGHDVLD

SEQ ID NO: 28031 - protein, 9 aa, synthetic construct
GGEGNDIVN

SEQ ID NO: 28032 - protein, 9 aa, synthetic construct
GGEGADTVD

SEQ ID NO: 28033 - protein, 9 aa, synthetic construct
GGEGADILL

SEQ ID NO: 28034 - protein, 9 aa, synthetic construct
GGEGDDFML

SEQ ID NO: 28035 - protein, 9 aa, synthetic construct
GGEGHDVLN

SEQ ID NO: 28036 - protein, 9 aa, synthetic construct
GGEGDDFMS

SEQ ID NO: 28037 - protein, 9 aa, synthetic construct
GGEGFDLVA

SEQ ID NO: 28038 - protein, 9 aa, synthetic construct
GGEGHDVLK

SEQ ID NO: 28039 - protein, 9 aa, synthetic construct
GGEGADILS

SEQ ID NO: 28040 - protein, 9 aa, synthetic construct
GGEGEDFIR

SEQ ID NO: 28041 - protein, 9 aa, synthetic construct
GGEGMDRLT

SEQ ID NO: 28042 - protein, 9 aa, synthetic construct
GGEGHDVLI

SEQ ID NO: 28043 - protein, 9 aa, synthetic construct
GGEGPDRLD

SEQ ID NO: 28044 - protein, 9 aa, synthetic construct
GGEGNDIVL

SEQ ID NO: 28045 - protein, 9 aa, synthetic construct
GGEGMDRID

SEQ ID NO: 28046 - protein, 9 aa, synthetic construct
GGEGHDVLE

SEQ ID NO: 28047 - protein, 9 aa, synthetic construct
GGEGIDRLA

SEQ ID NO: 28048 - protein, 9 aa, synthetic construct
GGEGHDTMR

SEQ ID NO: 28049 - protein, 9 aa, synthetic construct
GGEGQDALQ

SEQ ID NO: 28050 - protein, 9 aa, synthetic construct
GGEGNDIVQ

SEQ ID NO: 28051 - protein, 9 aa, synthetic construct
GGEGFDYLE

SEQ ID NO: 28052 - protein, 9 aa, synthetic construct
GGEGHDTLM

SEQ ID NO: 28053 - protein, 9 aa, synthetic construct
GGEGNDYMN

SEQ ID NO: 28054 - protein, 9 aa, synthetic construct
GGEGEDEVL

SEQ ID NO: 28055 - protein, 9 aa, synthetic construct
GGEGADIMR

SEQ ID NO: 28056 - protein, 9 aa, synthetic construct
GGEGGDAIH

SEQ ID NO: 28057 - protein, 9 aa, synthetic construct
GGEGMDLLI

SEQ ID NO: 28058 - protein, 9 aa, synthetic construct
GGEGADIVG

SEQ ID NO: 28059 - protein, 9 aa, synthetic construct
GGEGFDLAD

SEQ ID NO: 28060 - protein, 9 aa, synthetic construct
GGEGIDSLF

SEQ ID NO: 28061 - protein, 9 aa, synthetic construct
GGEGDDQLQ

SEQ ID NO: 28062 - protein, 9 aa, synthetic construct
GGEGDDQLN

SEQ ID NO: 28063 - protein, 9 aa, synthetic construct
GGEGIDSLN

SEQ ID NO: 28064 - protein, 9 aa, synthetic construct
GGEGDDEVN

SEQ ID NO: 28065 - protein, 9 aa, synthetic construct
GGEGADWLR

SEQ ID NO: 28066 - protein, 9 aa, synthetic construct
GGEGNDHLQ

SEQ ID NO: 28067 - protein, 9 aa, synthetic construct
GGEGADIME

SEQ ID NO: 28068 - protein, 9 aa, synthetic construct
GGEGCDTLY

SEQ ID NO: 28069 - protein, 9 aa, synthetic construct
GGEGMDLVD

SEQ ID NO: 28070 - protein, 9 aa, synthetic construct
GGEGNDIVS

SEQ ID NO: 28071 - protein, 9 aa, synthetic construct
GGEGPDEIY

SEQ ID NO: 28072 - protein, 9 aa, synthetic construct
GGEGNDIVT

SEQ ID NO: 28073 - protein, 9 aa, synthetic construct
GGEGIDRLV

SEQ ID NO: 28074 - protein, 9 aa, synthetic construct
GGEGEDEVY

SEQ ID NO: 28075 - protein, 9 aa, synthetic construct
GGEGADIMD

SEQ ID NO: 28076 - protein, 9 aa, synthetic construct
GGEGNDIVY

SEQ ID NO: 28077 - protein, 9 aa, synthetic construct
GGEGNDIYL

SEQ ID NO: 28078 - protein, 9 aa, synthetic construct
GGEGEDIIR

SEQ ID NO: 28079 - protein, 9 aa, synthetic construct
GGEGNDYVY

SEQ ID NO: 28080 - protein, 9 aa, synthetic construct
GGEGHDTLW

SEQ ID NO: 28081 - protein, 9 aa, synthetic construct
GGEGDDQLV

SEQ ID NO: 28082 - protein, 9 aa, synthetic construct
GGEGDDFVF

SEQ ID NO: 28083 - protein, 9 aa, synthetic construct
GGEGDDFVH

SEQ ID NO: 28084 - protein, 9 aa, synthetic construct
GGEGFDLVS

SEQ ID NO: 28085 - protein, 9 aa, synthetic construct
GGEGPDRLL

SEQ ID NO: 28086 - protein, 9 aa, synthetic construct
GGEGFDQAN

SEQ ID NO: 28087 - protein, 9 aa, synthetic construct
GGEGHDVLR

SEQ ID NO: 28088 - protein, 9 aa, synthetic construct
GGEGIDLVV

SEQ ID NO: 28089 - protein, 9 aa, synthetic construct
GGEGDDRAW

SEQ ID NO: 28090 - protein, 9 aa, synthetic construct
GGEGPDTLL

SEQ ID NO: 28091 - protein, 9 aa, synthetic construct
GGEGPDTLH

SEQ ID NO: 28092 - protein, 9 aa, synthetic construct
GGEGADIIG

SEQ ID NO: 28093 - protein, 9 aa, synthetic construct
GGEGPDTLD

SEQ ID NO: 28094 - protein, 9 aa, synthetic construct
GGEGHDWIF

SEQ ID NO: 28095 - protein, 9 aa, synthetic construct
GGEGIDMAA

SEQ ID NO: 28096 - protein, 9 aa, synthetic construct
GGEGDDFAS

SEQ ID NO: 28097 - protein, 9 aa, synthetic construct
GGEGHDVYR

SEQ ID NO: 28098 - protein, 9 aa, synthetic construct
GGEGHDVVL

SEQ ID NO: 28099 - protein, 9 aa, synthetic construct
GGEGHDVVE

SEQ ID NO: 28100 - protein, 9 aa, synthetic construct
GGEGNDRMY

SEQ ID NO: 28101 - protein, 9 aa, synthetic construct
GGEGIDMLL

SEQ ID NO: 28102 - protein, 9 aa, synthetic construct
GGEGIDNIF

SEQ ID NO: 28103 - protein, 9 aa, synthetic construct
GGEGDDFFA

SEQ ID NO: 28104 - protein, 9 aa, synthetic construct
GGEGADYVY

SEQ ID NO: 28105 - protein, 9 aa, synthetic construct
GGEGIDLMW

SEQ ID NO: 28106 - protein, 9 aa, synthetic construct
GGEGEDFLD

SEQ ID NO: 28107 - protein, 9 aa, synthetic construct
GGEGNDIMG

SEQ ID NO: 28108 - protein, 9 aa, synthetic construct
GGEGADIFT

SEQ ID NO: 28109 - protein, 9 aa, synthetic construct
GGEGNDIMI

SEQ ID NO: 28110 - protein, 9 aa, synthetic construct
GGEGFDVYR

SEQ ID NO: 28111 - protein, 9 aa, synthetic construct
GGEGGDSIL

SEQ ID NO: 28112 - protein, 9 aa, synthetic construct
GGEGADSFE

SEQ ID NO: 28113 - protein, 9 aa, synthetic construct
GGEGQDALD

SEQ ID NO: 28114 - protein, 9 aa, synthetic construct
GGEGDDRAY

SEQ ID NO: 28115 - protein, 9 aa, synthetic construct
GGEGQDAAV

SEQ ID NO: 28116 - protein, 9 aa, synthetic construct
GGEGPDVFV

SEQ ID NO: 28117 - protein, 9 aa, synthetic construct
GGEGPDTLY

SEQ ID NO: 28118 - protein, 9 aa, synthetic construct
GGEGNDAII

SEQ ID NO: 28119 - protein, 9 aa, synthetic construct
GGEGDDFLT

SEQ ID NO: 28120 - protein, 9 aa, synthetic construct
GGEGDDRFD

SEQ ID NO: 28121 - protein, 9 aa, synthetic construct
GGEGDDRAQ

SEQ ID NO: 28122 - protein, 9 aa, synthetic construct
GGEGNDIMQ

SEQ ID NO: 28123 - protein, 9 aa, synthetic construct
GGEGNDIMS

SEQ ID NO: 28124 - protein, 9 aa, synthetic construct
GGEGPDSLR

SEQ ID NO: 28125 - protein, 9 aa, synthetic construct
GGEGFDQVD

SEQ ID NO: 28126 - protein, 9 aa, synthetic construct
GGEGFDQLV

SEQ ID NO: 28127 - protein, 9 aa, synthetic construct
GGEGDDIYR

SEQ ID NO: 28128 - protein, 9 aa, synthetic construct
GGEGNDHVD

SEQ ID NO: 28129 - protein, 9 aa, synthetic construct
GGEGIDNLS

SEQ ID NO: 28130 - protein, 9 aa, synthetic construct
GGEGNDAIR

SEQ ID NO: 28131 - protein, 9 aa, synthetic construct
GGEGFDQID

SEQ ID NO: 28132 - protein, 9 aa, synthetic construct
GGEGGDSIT

SEQ ID NO: 28133 - protein, 9 aa, synthetic construct
GGEGADSFA

SEQ ID NO: 28134 - protein, 9 aa, synthetic construct
GGEGNDHMY

SEQ ID NO: 28135 - protein, 9 aa, synthetic construct
GGEGDDQMT

SEQ ID NO: 28136 - protein, 9 aa, synthetic construct
GGEGPDRLM

SEQ ID NO: 28137 - protein, 9 aa, synthetic construct
GGEGNDIVK

SEQ ID NO: 28138 - protein, 9 aa, synthetic construct
GGEGDDIYQ

SEQ ID NO: 28139 - protein, 9 aa, synthetic construct
GGEGADILG

SEQ ID NO: 28140 - protein, 9 aa, synthetic construct
GGEGDDEVW

SEQ ID NO: 28141 - protein, 9 aa, synthetic construct
GGEGHDVMR

SEQ ID NO: 28142 - protein, 9 aa, synthetic construct
GGEGDDSLR

SEQ ID NO: 28143 - protein, 9 aa, synthetic construct
GGEGDDRAD

SEQ ID NO: 28144 - protein, 9 aa, synthetic construct
GGEGNDRMT

SEQ ID NO: 28145 - protein, 9 aa, synthetic construct
GGEGMDSME

SEQ ID NO: 28146 - protein, 9 aa, synthetic construct
GGEGFDRLD

SEQ ID NO: 28147 - protein, 9 aa, synthetic construct
GGEGFDYAR

SEQ ID NO: 28148 - protein, 9 aa, synthetic construct
GGEGHDVLV

SEQ ID NO: 28149 - protein, 9 aa, synthetic construct
GGEGPDTIT

SEQ ID NO: 28150 - protein, 9 aa, synthetic construct
GGEGADSLG

SEQ ID NO: 28151 - protein, 9 aa, synthetic construct
GGEGDDQYV

SEQ ID NO: 28152 - protein, 9 aa, synthetic construct
GGEGDDQYI

SEQ ID NO: 28153 - protein, 9 aa, synthetic construct
GGEGADSFD

SEQ ID NO: 28154 - protein, 9 aa, synthetic construct
GGEGNDIVF

SEQ ID NO: 28155 - protein, 9 aa, synthetic construct
GGEGIDNLQ

SEQ ID NO: 28156 - protein, 9 aa, synthetic construct
GGEGFDYAS

SEQ ID NO: 28157 - protein, 9 aa, synthetic construct
GGEGCDTLK

SEQ ID NO: 28158 - protein, 9 aa, synthetic construct
GGEGDDNIE

SEQ ID NO: 28159 - protein, 9 aa, synthetic construct
GGEGNDFLG

SEQ ID NO: 28160 - protein, 9 aa, synthetic construct
GGEGNDPIY

SEQ ID NO: 28161 - protein, 9 aa, synthetic construct
GGEGNDEIN

SEQ ID NO: 28162 - protein, 9 aa, synthetic construct
GGEGNDNVS

SEQ ID NO: 28163 - protein, 9 aa, synthetic construct
GGEGKDRLE

SEQ ID NO: 28164 - protein, 9 aa, synthetic construct
GGEGADQIT

SEQ ID NO: 28165 - protein, 9 aa, synthetic construct
GGEGGDYLF

SEQ ID NO: 28166 - protein, 9 aa, synthetic construct
GGEGNDAVD

SEQ ID NO: 28167 - protein, 9 aa, synthetic construct
GGEGKDRLL

SEQ ID NO: 28168 - protein, 9 aa, synthetic construct
GGEGDDVVF

SEQ ID NO: 28169 - protein, 9 aa, synthetic construct
GGEGNDQAR

SEQ ID NO: 28170 - protein, 9 aa, synthetic construct
GGEGADRLR

SEQ ID NO: 28171 - protein, 9 aa, synthetic construct
GGEGGDYIF

SEQ ID NO: 28172 - protein, 9 aa, synthetic construct
GGEGKDVVN

SEQ ID NO: 28173 - protein, 9 aa, synthetic construct
GGEGDDLIN

SEQ ID NO: 28174 - protein, 9 aa, synthetic construct
GGEGNDEIE

SEQ ID NO: 28175 - protein, 9 aa, synthetic construct
GGEGKDRLA

SEQ ID NO: 28176 - protein, 9 aa, synthetic construct
GGEGADTIA

SEQ ID NO: 28177 - protein, 9 aa, synthetic construct
GGEGGDLLS

SEQ ID NO: 28178 - protein, 9 aa, synthetic construct
GGEGNDNLW

SEQ ID NO: 28179 - protein, 9 aa, synthetic construct
GGEGADQIS

SEQ ID NO: 28180 - protein, 9 aa, synthetic construct
GGEGGDLML

SEQ ID NO: 28181 - protein, 9 aa, synthetic construct
GGEGADVLK

SEQ ID NO: 28182 - protein, 9 aa, synthetic construct
GGEGDDIVS

SEQ ID NO: 28183 - protein, 9 aa, synthetic construct
GGEGNDNLV

SEQ ID NO: 28184 - protein, 9 aa, synthetic construct
GGEGEDRLI

SEQ ID NO: 28185 - protein, 9 aa, synthetic construct
GGEGNDELE

SEQ ID NO: 28186 - protein, 9 aa, synthetic construct
GGEGNDNVA

SEQ ID NO: 28187 - protein, 9 aa, synthetic construct
GGEGGDTLA

SEQ ID NO: 28188 - protein, 9 aa, synthetic construct
GGEGGDYLN

SEQ ID NO: 28189 - protein, 9 aa, synthetic construct
GGEGNDELA

SEQ ID NO: 28190 - protein, 9 aa, synthetic construct
GGEGDDIVR

SEQ ID NO: 28191 - protein, 9 aa, synthetic construct
GGEGNDEIW

SEQ ID NO: 28192 - protein, 9 aa, synthetic construct
GGEGNDEIR

SEQ ID NO: 28193 - protein, 9 aa, synthetic construct
GGEGADTFY

SEQ ID NO: 28194 - protein, 9 aa, synthetic construct
GGEGDDLIH

SEQ ID NO: 28195 - protein, 9 aa, synthetic construct
GGEGKDRLV

SEQ ID NO: 28196 - protein, 9 aa, synthetic construct
GGEGNDDVA

SEQ ID NO: 28197 - protein, 9 aa, synthetic construct
GGEGEDRLL

SEQ ID NO: 28198 - protein, 9 aa, synthetic construct
GGEGNDTLC

SEQ ID NO: 28199 - protein, 9 aa, synthetic construct
GGEGNDDVR

SEQ ID NO: 28200 - protein, 9 aa, synthetic construct
GGEGDDVVV

SEQ ID NO: 28201 - protein, 9 aa, synthetic construct
GGEGADRLM

SEQ ID NO: 28202 - protein, 9 aa, synthetic construct
GGEGGDWLL

SEQ ID NO: 28203 - protein, 9 aa, synthetic construct
GGEGADTFM

SEQ ID NO: 28204 - protein, 9 aa, synthetic construct
GGEGGDLMN

SEQ ID NO: 28205 - protein, 9 aa, synthetic construct
GGEGDDVYA

SEQ ID NO: 28206 - protein, 9 aa, synthetic construct
GGEGKDSLS

SEQ ID NO: 28207 - protein, 9 aa, synthetic construct
GGEGDDDVF

SEQ ID NO: 28208 - protein, 9 aa, synthetic construct
GGEGKDSVR

SEQ ID NO: 28209 - protein, 9 aa, synthetic construct
GGEGGDVYV

SEQ ID NO: 28210 - protein, 9 aa, synthetic construct
GGEGKDVLQ

SEQ ID NO: 28211 - protein, 9 aa, synthetic construct
GGEGGDTLK

SEQ ID NO: 28212 - protein, 9 aa, synthetic construct
GGEGDDVVS

SEQ ID NO: 28213 - protein, 9 aa, synthetic construct
GGEGKDVLS

SEQ ID NO: 28214 - protein, 9 aa, synthetic construct
GGEGKDSFV

SEQ ID NO: 28215 - protein, 9 aa, synthetic construct
GGEGADVLH

SEQ ID NO: 28216 - protein, 9 aa, synthetic construct
GGEGADRLQ

SEQ ID NO: 28217 - protein, 9 aa, synthetic construct
GGEGKDVLT

SEQ ID NO: 28218 - protein, 9 aa, synthetic construct
GGEGGDTLI

SEQ ID NO: 28219 - protein, 9 aa, synthetic construct
GGEGGDNLE

SEQ ID NO: 28220 - protein, 9 aa, synthetic construct
GGEGDDVVH

SEQ ID NO: 28221 - protein, 9 aa, synthetic construct
GGEGDDLFT

SEQ ID NO: 28222 - protein, 9 aa, synthetic construct
GGEGKDSFL

SEQ ID NO: 28223 - protein, 9 aa, synthetic construct
GGEGADTFT

SEQ ID NO: 28224 - protein, 9 aa, synthetic construct
GGEGNDQID

SEQ ID NO: 28225 - protein, 9 aa, synthetic construct
GGEGDDLIE

SEQ ID NO: 28226 - protein, 9 aa, synthetic construct
GGEGEDTLD

SEQ ID NO: 28227 - protein, 9 aa, synthetic construct
GGEGKDRVK

SEQ ID NO: 28228 - protein, 9 aa, synthetic construct
GGEGGDLLT

SEQ ID NO: 28229 - protein, 9 aa, synthetic construct
GGEGDDYIL

SEQ ID NO: 28230 - protein, 9 aa, synthetic construct
GGEGADLIV

SEQ ID NO: 28231 - protein, 9 aa, synthetic construct
GGEGGDLLG

SEQ ID NO: 28232 - protein, 9 aa, synthetic construct
GGEGHDDLY

SEQ ID NO: 28233 - protein, 9 aa, synthetic construct
GGEGNDRII

SEQ ID NO: 28234 - protein, 9 aa, synthetic construct
GGEGEDTVF

SEQ ID NO: 28235 - protein, 9 aa, synthetic construct
GGEGEDRLA

SEQ ID NO: 28236 - protein, 9 aa, synthetic construct
GGEGKDRFV

SEQ ID NO: 28237 - protein, 9 aa, synthetic construct
GGEGNDNLD

SEQ ID NO: 28238 - protein, 9 aa, synthetic construct
GGEGNDTMY

SEQ ID NO: 28239 - protein, 9 aa, synthetic construct
GGEGDDIIR

SEQ ID NO: 28240 - protein, 9 aa, synthetic construct
GGEGDDKLN

SEQ ID NO: 28241 - protein, 9 aa, synthetic construct
GGEGGDLLI

SEQ ID NO: 28242 - protein, 9 aa, synthetic construct
GGEGEDTVD

SEQ ID NO: 28243 - protein, 9 aa, synthetic construct
GGEGNDELM

SEQ ID NO: 28244 - protein, 9 aa, synthetic construct
GGEGDDEAG

SEQ ID NO: 28245 - protein, 9 aa, synthetic construct
GGEGDDVMA

SEQ ID NO: 28246 - protein, 9 aa, synthetic construct
GGEGKDQLV

SEQ ID NO: 28247 - protein, 9 aa, synthetic construct
GGEGGDTIT

SEQ ID NO: 28248 - protein, 9 aa, synthetic construct
GGEGGDLLQ

SEQ ID NO: 28249 - protein, 9 aa, synthetic construct
GGEGDDYIW

SEQ ID NO: 28250 - protein, 9 aa, synthetic construct
GGEGNDNIF

SEQ ID NO: 28251 - protein, 9 aa, synthetic construct
GGEGADTIR

SEQ ID NO: 28252 - protein, 9 aa, synthetic construct
GGEGKDQLD

SEQ ID NO: 28253 - protein, 9 aa, synthetic construct
GGEGADNIT

SEQ ID NO: 28254 - protein, 9 aa, synthetic construct
GGEGDDVIW

SEQ ID NO: 28255 - protein, 9 aa, synthetic construct
GGEGDDVIY

SEQ ID NO: 28256 - protein, 9 aa, synthetic construct
GGEGNDNII

SEQ ID NO: 28257 - protein, 9 aa, synthetic construct
GGEGKDYVE

SEQ ID NO: 28258 - protein, 9 aa, synthetic construct
GGEGEDQLV

SEQ ID NO: 28259 - protein, 9 aa, synthetic construct
GGEGHDELQ

SEQ ID NO: 28260 - protein, 9 aa, synthetic construct
GGEGADNLD

SEQ ID NO: 28261 - protein, 9 aa, synthetic construct
GGEGGDTIQ

SEQ ID NO: 28262 - protein, 9 aa, synthetic construct
GGEGDDIII

SEQ ID NO: 28263 - protein, 9 aa, synthetic construct
GGEGHDEIY

SEQ ID NO: 28264 - protein, 9 aa, synthetic construct
GGEGADNLN

SEQ ID NO: 28265 - protein, 9 aa, synthetic construct
GGEGDDIIW

SEQ ID NO: 28266 - protein, 9 aa, synthetic construct
GGEGDDKLR

SEQ ID NO: 28267 - protein, 9 aa, synthetic construct
GGEGADQIL

SEQ ID NO: 28268 - protein, 9 aa, synthetic construct
GGEGHDAID

SEQ ID NO: 28269 - protein, 9 aa, synthetic construct
GGEGDDYIN

SEQ ID NO: 28270 - protein, 9 aa, synthetic construct
GGEGNDNLN

SEQ ID NO: 28271 - protein, 9 aa, synthetic construct
GGEGNDELK

SEQ ID NO: 28272 - protein, 9 aa, synthetic construct
GGEGNDELI

SEQ ID NO: 28273 - protein, 9 aa, synthetic construct
GGEGADTIH

SEQ ID NO: 28274 - protein, 9 aa, synthetic construct
GGEGKDRIT

SEQ ID NO: 28275 - protein, 9 aa, synthetic construct
GGEGEDTLW

SEQ ID NO: 28276 - protein, 9 aa, synthetic construct
GGEGDDVVA

SEQ ID NO: 28277 - protein, 9 aa, synthetic construct
GGEGKDVYI

SEQ ID NO: 28278 - protein, 9 aa, synthetic construct
GGEGNDRFY

SEQ ID NO: 28279 - protein, 9 aa, synthetic construct
GGEGEDTLM

SEQ ID NO: 28280 - protein, 9 aa, synthetic construct
GGEGGDYYG

SEQ ID NO: 28281 - protein, 9 aa, synthetic construct
GGEGEDTLL

SEQ ID NO: 28282 - protein, 9 aa, synthetic construct
GGEGNDTMG

SEQ ID NO: 28283 - protein, 9 aa, synthetic construct
GGEGGDTIY

SEQ ID NO: 28284 - protein, 9 aa, synthetic construct
GGEGDDVMR

SEQ ID NO: 28285 - protein, 9 aa, synthetic construct
GGEGNDRIA

SEQ ID NO: 28286 - protein, 9 aa, synthetic construct
GGEGDDVMH

SEQ ID NO: 28287 - protein, 9 aa, synthetic construct
GGEGKDRIR

SEQ ID NO: 28288 - protein, 9 aa, synthetic construct
GGEGDDKLS

SEQ ID NO: 28289 - protein, 9 aa, synthetic construct
GGEGNDTMR

SEQ ID NO: 28290 - protein, 9 aa, synthetic construct
GGEGDDAVC

SEQ ID NO: 28291 - protein, 9 aa, synthetic construct
GGEGEDTLT

SEQ ID NO: 28292 - protein, 9 aa, synthetic construct
GGEGKDXIS

SEQ ID NO: 28293 - protein, 9 aa, synthetic construct
GGEGNDTMS

SEQ ID NO: 28294 - protein, 9 aa, synthetic construct
GGEGADQFA

SEQ ID NO: 28295 - protein, 9 aa, synthetic construct
GGEGADQAG

SEQ ID NO: 28296 - protein, 9 aa, synthetic construct
GGEGADNYY

SEQ ID NO: 28297 - protein, 9 aa, synthetic construct
GGEGNDNLH

SEQ ID NO: 28298 - protein, 9 aa, synthetic construct
GGEGADNLS

SEQ ID NO: 28299 - protein, 9 aa, synthetic construct
GGEGGDQLT

SEQ ID NO: 28300 - protein, 9 aa, synthetic construct
GGEGKDTAK

SEQ ID NO: 28301 - protein, 9 aa, synthetic construct
GGEGADQLV

SEQ ID NO: 28302 - protein, 9 aa, synthetic construct
GGEGNDQLV

SEQ ID NO: 28303 - protein, 9 aa, synthetic construct
GGEGGDTVR

SEQ ID NO: 28304 - protein, 9 aa, synthetic construct
GGEGDDWIY

SEQ ID NO: 28305 - protein, 9 aa, synthetic construct
GGEGDDYAE

SEQ ID NO: 28306 - protein, 9 aa, synthetic construct
GGEGADSVL

SEQ ID NO: 28307 - protein, 9 aa, synthetic construct
GGEGADSVF

SEQ ID NO: 28308 - protein, 9 aa, synthetic construct
GGEGNDRAS

SEQ ID NO: 28309 - protein, 9 aa, synthetic construct
GGEGADRIN

SEQ ID NO: 28310 - protein, 9 aa, synthetic construct
GGEGKDTVK

SEQ ID NO: 28311 - protein, 9 aa, synthetic construct
GGEGGDTMI

SEQ ID NO: 28312 - protein, 9 aa, synthetic construct
GGEGADRIQ

SEQ ID NO: 28313 - protein, 9 aa, synthetic construct
GGEGNDTIG

SEQ ID NO: 28314 - protein, 9 aa, synthetic construct
GGEGNDAYY

SEQ ID NO: 28315 - protein, 9 aa, synthetic construct
GGEGKDTVT

SEQ ID NO: 28316 - protein, 9 aa, synthetic construct
GGEGADVFT

SEQ ID NO: 28317 - protein, 9 aa, synthetic construct
GGEGEDSIS

SEQ ID NO: 28318 - protein, 9 aa, synthetic construct
GGEGDDWID

SEQ ID NO: 28319 - protein, 9 aa, synthetic construct
GGEGNDQIK

SEQ ID NO: 28320 - protein, 9 aa, synthetic construct
GGEGDDWIA

SEQ ID NO: 28321 - protein, 9 aa, synthetic construct
GGEGGDVFI

SEQ ID NO: 28322 - protein, 9 aa, synthetic construct
GGEGDDYFT

SEQ ID NO: 28323 - protein, 9 aa, synthetic construct
GGEGADTAF

SEQ ID NO: 28324 - protein, 9 aa, synthetic construct
GGEGEDRLT

SEQ ID NO: 28325 - protein, 9 aa, synthetic construct
GGEGADRIL

SEQ ID NO: 28326 - protein, 9 aa, synthetic construct
GGEGGDVFD

SEQ ID NO: 28327 - protein, 9 aa, synthetic construct
GGEGDDIMV

SEQ ID NO: 28328 - protein, 9 aa, synthetic construct
GGEGEDSLA

SEQ ID NO: 28329 - protein, 9 aa, synthetic construct
GGEGKDVLA

SEQ ID NO: 28330 - protein, 9 aa, synthetic construct
GGEGNDTFK

SEQ ID NO: 28331 - protein, 9 aa, synthetic construct
GGEGADSVT

SEQ ID NO: 28332 - protein, 9 aa, synthetic construct
GGEGGDVAI

SEQ ID NO: 28333 - protein, 9 aa, synthetic construct
GGEGGDTYY

SEQ ID NO: 28334 - protein, 9 aa, synthetic construct
GGEGDDYAS

SEQ ID NO: 28335 - protein, 9 aa, synthetic construct
GGEGKDVIY

SEQ ID NO: 28336 - protein, 9 aa, synthetic construct
GGEGDDWLG

SEQ ID NO: 28337 - protein, 9 aa, synthetic construct
GGEGEDRLY

SEQ ID NO: 28338 - protein, 9 aa, synthetic construct
GGEGADSML

SEQ ID NO: 28339 - protein, 9 aa, synthetic construct
GGEGDDWLR

SEQ ID NO: 28340 - protein, 9 aa, synthetic construct
GGEGNDQVF

SEQ ID NO: 28341 - protein, 9 aa, synthetic construct
GGEGGDTLS

SEQ ID NO: 28342 - protein, 9 aa, synthetic construct
GGEGDDWMS

SEQ ID NO: 28343 - protein, 9 aa, synthetic construct
GGEGNDQVY

SEQ ID NO: 28344 - protein, 9 aa, synthetic construct
GGEGDDWLS

SEQ ID NO: 28345 - protein, 9 aa, synthetic construct
GGEGNDRAE

SEQ ID NO: 28346 - protein, 9 aa, synthetic construct
GGEGDDAMS

SEQ ID NO: 28347 - protein, 9 aa, synthetic construct
GGEGNDRAG

SEQ ID NO: 28348 - protein, 9 aa, synthetic construct
GGEGKDVFR

SEQ ID NO: 28349 - protein, 9 aa, synthetic construct
GGEGDDWMK

SEQ ID NO: 28350 - protein, 9 aa, synthetic construct
GGEGEDRVS

SEQ ID NO: 28351 - protein, 9 aa, synthetic construct
GGEGNDRAL

SEQ ID NO: 28352 - protein, 9 aa, synthetic construct
GGEGADSMS

SEQ ID NO: 28353 - protein, 9 aa, synthetic construct
GGEGDDWLQ

SEQ ID NO: 28354 - protein, 9 aa, synthetic construct
GGEGKDVFI

SEQ ID NO: 28355 - protein, 9 aa, synthetic construct
GGEGNDDID

SEQ ID NO: 28356 - protein, 9 aa, synthetic construct
GGEGNDQMY

SEQ ID NO: 28357 - protein, 9 aa, synthetic construct
GGEGEDSII

SEQ ID NO: 28358 - protein, 9 aa, synthetic construct
GGEGGDTLY

SEQ ID NO: 28359 - protein, 9 aa, synthetic construct
GGEGADRIT

SEQ ID NO: 28360 - protein, 9 aa, synthetic construct
GGEGNDQMW

SEQ ID NO: 28361 - protein, 9 aa, synthetic construct
GGEGNDDIF

SEQ ID NO: 28362 - protein, 9 aa, synthetic construct
GGEGNDQMT

SEQ ID NO: 28363 - protein, 9 aa, synthetic construct
GGEGGDTME

SEQ ID NO: 28364 - protein, 9 aa, synthetic construct
GGEGKDTYV

SEQ ID NO: 28365 - protein, 9 aa, synthetic construct
GGEGNDQMN

SEQ ID NO: 28366 - protein, 9 aa, synthetic construct
GGEGDDWVA

SEQ ID NO: 28367 - protein, 9 aa, synthetic construct
GGEGDDWLH

SEQ ID NO: 28368 - protein, 9 aa, synthetic construct
GGEGNDQMI

SEQ ID NO: 28369 - protein, 9 aa, synthetic construct
GGEGNDTFM

SEQ ID NO: 28370 - protein, 9 aa, synthetic construct
GGEGADRIF

SEQ ID NO: 28371 - protein, 9 aa, synthetic construct
GGEGADRIE

SEQ ID NO: 28372 - protein, 9 aa, synthetic construct
GGEGKDTLT

SEQ ID NO: 28373 - protein, 9 aa, synthetic construct
GGEGEDTID

SEQ ID NO: 28374 - protein, 9 aa, synthetic construct
GGEGADTFF

SEQ ID NO: 28375 - protein, 9 aa, synthetic construct
GGEGADVFL

SEQ ID NO: 28376 - protein, 9 aa, synthetic construct
GGEGADQMY

SEQ ID NO: 28377 - protein, 9 aa, synthetic construct
GGEGDDLAS

SEQ ID NO: 28378 - protein, 9 aa, synthetic construct
GGEGNDQIW

SEQ ID NO: 28379 - protein, 9 aa, synthetic construct
GGEGGDTLL

SEQ ID NO: 28380 - protein, 9 aa, synthetic construct
GGEGNDDLH

SEQ ID NO: 28381 - protein, 9 aa, synthetic construct
GGEGDDYFV

SEQ ID NO: 28382 - protein, 9 aa, synthetic construct
GGEGADTFD

SEQ ID NO: 28383 - protein, 9 aa, synthetic construct
GGEGDDVYY

SEQ ID NO: 28384 - protein, 9 aa, synthetic construct
GGEGDDLAQ

SEQ ID NO: 28385 - protein, 9 aa, synthetic construct
GGEGKDTIH

SEQ ID NO: 28386 - protein, 9 aa, synthetic construct
GGEGADVIT

SEQ ID NO: 28387 - protein, 9 aa, synthetic construct
GGEGGDTLR

SEQ ID NO: 28388 - protein, 9 aa, synthetic construct
GGEGDDLAY

SEQ ID NO: 28389 - protein, 9 aa, synthetic construct
GGEGADTFG

SEQ ID NO: 28390 - protein, 9 aa, synthetic construct
GGEGGDVML

SEQ ID NO: 28391 - protein, 9 aa, synthetic construct
GGEGADQMS

SEQ ID NO: 28392 - protein, 9 aa, synthetic construct
GGEGNDAVV

SEQ ID NO: 28393 - protein, 9 aa, synthetic construct
GGEGNDDLN

SEQ ID NO: 28394 - protein, 9 aa, synthetic construct
GGEGADQME

SEQ ID NO: 28395 - protein, 9 aa, synthetic construct
GGEGGDNLQ

SEQ ID NO: 28396 - protein, 9 aa, synthetic construct
GGEGNDTIW

SEQ ID NO: 28397 - protein, 9 aa, synthetic construct
GGEGDDLFD

SEQ ID NO: 28398 - protein, 9 aa, synthetic construct
GGEGKDTFL

SEQ ID NO: 28399 - protein, 9 aa, synthetic construct
GGEGDDDMG

SEQ ID NO: 28400 - protein, 9 aa, synthetic construct
GGEGADQLY

SEQ ID NO: 28401 - protein, 9 aa, synthetic construct
GGEGEDRLN

SEQ ID NO: 28402 - protein, 9 aa, synthetic construct
GGEGKDVLK

SEQ ID NO: 28403 - protein, 9 aa, synthetic construct
GGEGKDTAV

SEQ ID NO: 28404 - protein, 9 aa, synthetic construct
GGEGDDILM

SEQ ID NO: 28405 - protein, 9 aa, synthetic construct
GGEGADQVL

SEQ ID NO: 28406 - protein, 9 aa, synthetic construct
GGEGADQVS

SEQ ID NO: 28407 - protein, 9 aa, synthetic construct
GGEGNDDIR

SEQ ID NO: 28408 - protein, 9 aa, synthetic construct
GGEGDDKLW

SEQ ID NO: 28409 - protein, 9 aa, synthetic construct
GGEGGDNLY

SEQ ID NO: 28410 - protein, 9 aa, synthetic construct
GGEGGDVIV

SEQ ID NO: 28411 - protein, 9 aa, synthetic construct
GGEGADVFQ

SEQ ID NO: 28412 - protein, 9 aa, synthetic construct
GGEGGDVIT

SEQ ID NO: 28413 - protein, 9 aa, synthetic construct
GGEGKDTLN

SEQ ID NO: 28414 - protein, 9 aa, synthetic construct
GGEGGDVIN

SEQ ID NO: 28415 - protein, 9 aa, synthetic construct
GGEGADRID

SEQ ID NO: 28416 - protein, 9 aa, synthetic construct
GGEGKDTIQ

SEQ ID NO: 28417 - protein, 9 aa, synthetic construct
GGEGGDQLS

SEQ ID NO: 28418 - protein, 9 aa, synthetic construct
GGEGEDSLE

SEQ ID NO: 28419 - protein, 9 aa, synthetic construct
GGEGADTAI

SEQ ID NO: 28420 - protein, 9 aa, synthetic construct
GGEGNDAYL

SEQ ID NO: 28421 - protein, 9 aa, synthetic construct
GGEGNDAYM

SEQ ID NO: 28422 - protein, 9 aa, synthetic construct
GGEGADTAG

SEQ ID NO: 28423 - protein, 9 aa, synthetic construct
GGEGKDTLG

SEQ ID NO: 28424 - protein, 9 aa, synthetic construct
GGEGGDVLC

SEQ ID NO: 28425 - protein, 9 aa, synthetic construct
GGEGNDRFE

SEQ ID NO: 28426 - protein, 9 aa, synthetic construct
GGEGKDTIY

SEQ ID NO: 28427 - protein, 9 aa, synthetic construct
GGEGADSMF

SEQ ID NO: 28428 - protein, 9 aa, synthetic construct
GGEGADTAY

SEQ ID NO: 28429 - protein, 9 aa, synthetic construct
GGEGGDVLL

SEQ ID NO: 28430 - protein, 9 aa, synthetic construct
GGEGEDSLH

SEQ ID NO: 28431 - protein, 9 aa, synthetic construct
GGEGADVIA

SEQ ID NO: 28432 - protein, 9 aa, synthetic construct
GGEGDDKVT

SEQ ID NO: 28433 - protein, 9 aa, synthetic construct
GGEGADRFR

SEQ ID NO: 28434 - protein, 9 aa, synthetic construct
GGEGADRFI

SEQ ID NO: 28435 - protein, 9 aa, synthetic construct
GGEGADRFA

SEQ ID NO: 28436 - protein, 9 aa, synthetic construct
GGEGDDLAH

SEQ ID NO: 28437 - protein, 9 aa, synthetic construct
GGEGADQVY

SEQ ID NO: 28438 - protein, 9 aa, synthetic construct
GGEGEDTAN

SEQ ID NO: 28439 - protein, 9 aa, synthetic construct
GGEGDDILW

SEQ ID NO: 28440 - protein, 9 aa, synthetic construct
GGEGNDNIE

SEQ ID NO: 28441 - protein, 9 aa, synthetic construct
GGEGLDAIF

SEQ ID NO: 28442 - protein, 9 aa, synthetic construct
GGEGADNIQ

SEQ ID NO: 28443 - protein, 9 aa, synthetic construct
GGEGDDMLI

SEQ ID NO: 28444 - protein, 9 aa, synthetic construct
GGEGEDYAF

SEQ ID NO: 28445 - protein, 9 aa, synthetic construct
GGEGADLLW

SEQ ID NO: 28446 - protein, 9 aa, synthetic construct
GGEGDDMLL

SEQ ID NO: 28447 - protein, 9 aa, synthetic construct
GGEGADLMI

SEQ ID NO: 28448 - protein, 9 aa, synthetic construct
GGEGKDHLD

SEQ ID NO: 28449 - protein, 9 aa, synthetic construct
GGEGADTVI

SEQ ID NO: 28450 - protein, 9 aa, synthetic construct
GGEGDDIVV

SEQ ID NO: 28451 - protein, 9 aa, synthetic construct
GGEGDDTMV

SEQ ID NO: 28452 - protein, 9 aa, synthetic construct
GGEGGDTII

SEQ ID NO: 28453 - protein, 9 aa, synthetic construct
GGEGDDHMW

SEQ ID NO: 28454 - protein, 9 aa, synthetic construct
GGEGEDWLH

SEQ ID NO: 28455 - protein, 9 aa, synthetic construct
GGEGADVMI

SEQ ID NO: 28456 - protein, 9 aa, synthetic construct
GGEGGDILT

SEQ ID NO: 28457 - protein, 9 aa, synthetic construct
GGEGKDIIN

SEQ ID NO: 28458 - protein, 9 aa, synthetic construct
GGEGHDLLV

SEQ ID NO: 28459 - protein, 9 aa, synthetic construct
GGEGKDFVE

SEQ ID NO: 28460 - protein, 9 aa, synthetic construct
GGEGLDSAW

SEQ ID NO: 28461 - protein, 9 aa, synthetic construct
GGEGNDVMF

SEQ ID NO: 28462 - protein, 9 aa, synthetic construct
GGEGDDHMN

SEQ ID NO: 28463 - protein, 9 aa, synthetic construct
GGEGNDVMI

SEQ ID NO: 28464 - protein, 9 aa, synthetic construct
GGEGNDFIT

SEQ ID NO: 28465 - protein, 9 aa, synthetic construct
GGEGNDVMG

SEQ ID NO: 28466 - protein, 9 aa, synthetic construct
GGEGGDTIE

SEQ ID NO: 28467 - protein, 9 aa, synthetic construct
GGEGEDLLM

SEQ ID NO: 28468 - protein, 9 aa, synthetic construct
GGEGDDTMH

SEQ ID NO: 28469 - protein, 9 aa, synthetic construct
GGEGNDVMA

SEQ ID NO: 28470 - protein, 9 aa, synthetic construct
GGEGNDVME

SEQ ID NO: 28471 - protein, 9 aa, synthetic construct
GGEGLDTAV

SEQ ID NO: 28472 - protein, 9 aa, synthetic construct
GGEGLDTAS

SEQ ID NO: 28473 - protein, 9 aa, synthetic construct
GGEGHDLMY

SEQ ID NO: 28474 - protein, 9 aa, synthetic construct
GGEGNDVMD

SEQ ID NO: 28475 - protein, 9 aa, synthetic construct
GGEGNDLIT

SEQ ID NO: 28476 - protein, 9 aa, synthetic construct
GGEGKDIIY

SEQ ID NO: 28477 - protein, 9 aa, synthetic construct
GGEGNDVLW

SEQ ID NO: 28478 - protein, 9 aa, synthetic construct
GGEGLDTAD

SEQ ID NO: 28479 - protein, 9 aa, synthetic construct
GGEGDDHYV

SEQ ID NO: 28480 - protein, 9 aa, synthetic construct
GGEGDDMIA

SEQ ID NO: 28481 - protein, 9 aa, synthetic construct
GGEGDDTVV

SEQ ID NO: 28482 - protein, 9 aa, synthetic construct
GGEGDDHVY

SEQ ID NO: 28483 - protein, 9 aa, synthetic construct
GGEGKDILK

SEQ ID NO: 28484 - protein, 9 aa, synthetic construct
GGEGDDLYR

SEQ ID NO: 28485 - protein, 9 aa, synthetic construct
GGEGLDSIF

SEQ ID NO: 28486 - protein, 9 aa, synthetic construct
GGEGDDTYA

SEQ ID NO: 28487 - protein, 9 aa, synthetic construct
GGEGKDILA

SEQ ID NO: 28488 - protein, 9 aa, synthetic construct
GGEGADLMY

SEQ ID NO: 28489 - protein, 9 aa, synthetic construct
GGEGNDALH

SEQ ID NO: 28490 - protein, 9 aa, synthetic construct
GGEGEDVLN

SEQ ID NO: 28491 - protein, 9 aa, synthetic construct
GGEGNDALI

SEQ ID NO: 28492 - protein, 9 aa, synthetic construct
GGEGNDLLW

SEQ ID NO: 28493 - protein, 9 aa, synthetic construct
GGEGADLVD

SEQ ID NO: 28494 - protein, 9 aa, synthetic construct
GGEGDDYVA

SEQ ID NO: 28495 - protein, 9 aa, synthetic construct
GGEGDDHVF

SEQ ID NO: 28496 - protein, 9 aa, synthetic construct
GGEGDDYVE

SEQ ID NO: 28497 - protein, 9 aa, synthetic construct
GGEGLDSLD

SEQ ID NO: 28498 - protein, 9 aa, synthetic construct
GGEGDDHVE

SEQ ID NO: 28499 - protein, 9 aa, synthetic construct
GGEGNDTAN

SEQ ID NO: 28500 - protein, 9 aa, synthetic construct
GGEGEDAFL

SEQ ID NO: 28501 - protein, 9 aa, synthetic construct
GGEGEDVLT

SEQ ID NO: 28502 - protein, 9 aa, synthetic construct
GGEGCDVLE

SEQ ID NO: 28503 - protein, 9 aa, synthetic construct
GGEGLDSVR

SEQ ID NO: 28504 - protein, 9 aa, synthetic construct
GGEGHDLAS

SEQ ID NO: 28505 - protein, 9 aa, synthetic construct
GGEGHDLIV

SEQ ID NO: 28506 - protein, 9 aa, synthetic construct
GGEGDDHVA

SEQ ID NO: 28507 - protein, 9 aa, synthetic construct
GGEGGDKLD

SEQ ID NO: 28508 - protein, 9 aa, synthetic construct
GGEGEDVVF

SEQ ID NO: 28509 - protein, 9 aa, synthetic construct
GGEGDDTVA

SEQ ID NO: 28510 - protein, 9 aa, synthetic construct
GGEGADVII

SEQ ID NO: 28511 - protein, 9 aa, synthetic construct
GGEGKDFMS

SEQ ID NO: 28512 - protein, 9 aa, synthetic construct
GGEGDDTMD

SEQ ID NO: 28513 - protein, 9 aa, synthetic construct
GGEGNDVMY

SEQ ID NO: 28514 - protein, 9 aa, synthetic construct
GGEGNDVYG

SEQ ID NO: 28515 - protein, 9 aa, synthetic construct
GGEGKDALQ

SEQ ID NO: 28516 - protein, 9 aa, synthetic construct
GGEGNDVYH

SEQ ID NO: 28517 - protein, 9 aa, synthetic construct
GGEGNDALC

SEQ ID NO: 28518 - protein, 9 aa, synthetic construct
GGEGFDELS

SEQ ID NO: 28519 - protein, 9 aa, synthetic construct
GGEGKDDLH

SEQ ID NO: 28520 - protein, 9 aa, synthetic construct
GGEGDDNIF

SEQ ID NO: 28521 - protein, 9 aa, synthetic construct
GGEGNDVYF

SEQ ID NO: 28522 - protein, 9 aa, synthetic construct
GGEGDDMVS

SEQ ID NO: 28523 - protein, 9 aa, synthetic construct
GGEGFDELL

SEQ ID NO: 28524 - protein, 9 aa, synthetic construct
GGEGGDRID

SEQ ID NO: 28525 - protein, 9 aa, synthetic construct
GGEGLDTMM

SEQ ID NO: 28526 - protein, 9 aa, synthetic construct
GGEGADLLM

SEQ ID NO: 28527 - protein, 9 aa, synthetic construct
GGEGDDELA

SEQ ID NO: 28528 - protein, 9 aa, synthetic construct
GGEGKDDLQ

SEQ ID NO: 28529 - protein, 9 aa, synthetic construct
GGEGHDNLN

SEQ ID NO: 28530 - protein, 9 aa, synthetic construct
GGEGGDTFI

SEQ ID NO: 28531 - protein, 9 aa, synthetic construct
GGEGLDVAD

SEQ ID NO: 28532 - protein, 9 aa, synthetic construct
GGEGADLLH

SEQ ID NO: 28533 - protein, 9 aa, synthetic construct
GGEGDDNII

SEQ ID NO: 28534 - protein, 9 aa, synthetic construct
GGEGNDVYS

SEQ ID NO: 28535 - protein, 9 aa, synthetic construct
GGEGHDQIA

SEQ ID NO: 28536 - protein, 9 aa, synthetic construct
GGEGHDQIF

SEQ ID NO: 28537 - protein, 9 aa, synthetic construct
GGEGNDLFQ

SEQ ID NO: 28538 - protein, 9 aa, synthetic construct
GGEGHDQLD

SEQ ID NO: 28539 - protein, 9 aa, synthetic construct
GGEGDDIYD

SEQ ID NO: 28540 - protein, 9 aa, synthetic construct
GGEGDDNIR

SEQ ID NO: 28541 - protein, 9 aa, synthetic construct
GGEGDDNIS

SEQ ID NO: 28542 - protein, 9 aa, synthetic construct
GGEGHDQLF

SEQ ID NO: 28543 - protein, 9 aa, synthetic construct
GGEGKDALF

SEQ ID NO: 28544 - protein, 9 aa, synthetic construct
GGEGIDYVS

SEQ ID NO: 28545 - protein, 9 aa, synthetic construct
GGEGIDYLR

SEQ ID NO: 28546 - protein, 9 aa, synthetic construct
GGEGLDTMD

SEQ ID NO: 28547 - protein, 9 aa, synthetic construct
GGEGADLLN

SEQ ID NO: 28548 - protein, 9 aa, synthetic construct
GGEGNDLIR

SEQ ID NO: 28549 - protein, 9 aa, synthetic construct
GGEGLDTLD

SEQ ID NO: 28550 - protein, 9 aa, synthetic construct
GGEGEDLIW

SEQ ID NO: 28551 - protein, 9 aa, synthetic construct
GGEGDDHLR

SEQ ID NO: 28552 - protein, 9 aa, synthetic construct
GGEGADVMY

SEQ ID NO: 28553 - protein, 9 aa, synthetic construct
GGEGHDMLW

SEQ ID NO: 28554 - protein, 9 aa, synthetic construct
GGEGDDHLT

SEQ ID NO: 28555 - protein, 9 aa, synthetic construct
GGEGHDLVY

SEQ ID NO: 28556 - protein, 9 aa, synthetic construct
GGEGKDFLT

SEQ ID NO: 28557 - protein, 9 aa, synthetic construct
GGEGKDDLS

SEQ ID NO: 28558 - protein, 9 aa, synthetic construct
GGEGDDMLV

SEQ ID NO: 28559 - protein, 9 aa, synthetic construct
GGEGHDLVN

SEQ ID NO: 28560 - protein, 9 aa, synthetic construct
GGEGEDYID

SEQ ID NO: 28561 - protein, 9 aa, synthetic construct
GGEGGDIFA

SEQ ID NO: 28562 - protein, 9 aa, synthetic construct
GGEGLDTIL

SEQ ID NO: 28563 - protein, 9 aa, synthetic construct
GGEGNDFIX

SEQ ID NO: 28564 - protein, 9 aa, synthetic construct
GGEGHDNIR

SEQ ID NO: 28565 - protein, 9 aa, synthetic construct
GGEGGDTIA

SEQ ID NO: 28566 - protein, 9 aa, synthetic construct
GGEGADVYL

SEQ ID NO: 28567 - protein, 9 aa, synthetic construct
GGEGADWFA

SEQ ID NO: 28568 - protein, 9 aa, synthetic construct
GGEGNDVVF

SEQ ID NO: 28569 - protein, 9 aa, synthetic construct
GGEGEDYLT

SEQ ID NO: 28570 - protein, 9 aa, synthetic construct
GGEGHDNIY

SEQ ID NO: 28571 - protein, 9 aa, synthetic construct
GGEGEDYLV

SEQ ID NO: 28572 - protein, 9 aa, synthetic construct
GGEGNDVVN

SEQ ID NO: 28573 - protein, 9 aa, synthetic construct
GGEGKDELK

SEQ ID NO: 28574 - protein, 9 aa, synthetic construct
GGEGLDTLN

SEQ ID NO: 28575 - protein, 9 aa, synthetic construct
GGEGKDEIH

SEQ ID NO: 28576 - protein, 9 aa, synthetic construct
GGEGFDDLF

SEQ ID NO: 28577 - protein, 9 aa, synthetic construct
GGEGKDEID

SEQ ID NO: 28578 - protein, 9 aa, synthetic construct
GGEGNDLIC

SEQ ID NO: 28579 - protein, 9 aa, synthetic construct
GGEGLDTLY

SEQ ID NO: 28580 - protein, 9 aa, synthetic construct
GGEGHDNLF

SEQ ID NO: 28581 - protein, 9 aa, synthetic construct
GGEGKDIMV

SEQ ID NO: 28582 - protein, 9 aa, synthetic construct
GGEGADLVF

SEQ ID NO: 28583 - protein, 9 aa, synthetic construct
GGEGNDTVG

SEQ ID NO: 28584 - protein, 9 aa, synthetic construct
GGEGNDELV

SEQ ID NO: 28585 - protein, 9 aa, synthetic construct
GGEGNDMLD

SEQ ID NO: 28586 - protein, 9 aa, synthetic construct
GGEGADTVY

SEQ ID NO: 28587 - protein, 9 aa, synthetic construct
GGEGHDIFV

SEQ ID NO: 28588 - protein, 9 aa, synthetic construct
GGEGADTYF

SEQ ID NO: 28589 - protein, 9 aa, synthetic construct
GGEGLDLLI

SEQ ID NO: 28590 - protein, 9 aa, synthetic construct
GGEGDDAIT

SEQ ID NO: 28591 - protein, 9 aa, synthetic construct
GGEGHDIFQ

SEQ ID NO: 28592 - protein, 9 aa, synthetic construct
GGEGNDMIY

SEQ ID NO: 28593 - protein, 9 aa, synthetic construct
GGEGADSLM

SEQ ID NO: 28594 - protein, 9 aa, synthetic construct
GGEGNDMLT

SEQ ID NO: 28595 - protein, 9 aa, synthetic construct
GGEGHDIAY

SEQ ID NO: 28596 - protein, 9 aa, synthetic construct
GGEGNDTYE

SEQ ID NO: 28597 - protein, 9 aa, synthetic construct
GGEGLDLLD

SEQ ID NO: 28598 - protein, 9 aa, synthetic construct
GGEGNDMLV

SEQ ID NO: 28599 - protein, 9 aa, synthetic construct
GGEGADTIS

SEQ ID NO: 28600 - protein, 9 aa, synthetic construct
GGEGNDELW

SEQ ID NO: 28601 - protein, 9 aa, synthetic construct
GGEGEDVLH

SEQ ID NO: 28602 - protein, 9 aa, synthetic construct
GGEGNDVAE

SEQ ID NO: 28603 - protein, 9 aa, synthetic construct
GGEGLDLLS

SEQ ID NO: 28604 - protein, 9 aa, synthetic construct
GGEGNDVAF

SEQ ID NO: 28605 - protein, 9 aa, synthetic construct
GGEGDDIFY

SEQ ID NO: 28606 - protein, 9 aa, synthetic construct
GGEGNDEVD

SEQ ID NO: 28607 - protein, 9 aa, synthetic construct
GGEGNDLYL

SEQ ID NO: 28608 - protein, 9 aa, synthetic construct
GGEGHDILD

SEQ ID NO: 28609 - protein, 9 aa, synthetic construct
GGEGNDLYR

SEQ ID NO: 28610 - protein, 9 aa, synthetic construct
GGEGADMLQ

SEQ ID NO: 28611 - protein, 9 aa, synthetic construct
GGEGEDVAR

SEQ ID NO: 28612 - protein, 9 aa, synthetic construct
GGEGNDMAV

SEQ ID NO: 28613 - protein, 9 aa, synthetic construct
GGEGDDAIG

SEQ ID NO: 28614 - protein, 9 aa, synthetic construct
GGEGLDLLL

SEQ ID NO: 28615 - protein, 9 aa, synthetic construct
GGEGADMLL

SEQ ID NO: 28616 - protein, 9 aa, synthetic construct
GGEGNDMIS

SEQ ID NO: 28617 - protein, 9 aa, synthetic construct
GGEGLDKLT

SEQ ID NO: 28618 - protein, 9 aa, synthetic construct
GGEGKDMFV

SEQ ID NO: 28619 - protein, 9 aa, synthetic construct
GGEGDDVIK

SEQ ID NO: 28620 - protein, 9 aa, synthetic construct
GGEGNDRIK

SEQ ID NO: 28621 - protein, 9 aa, synthetic construct
GGEGLDILI

SEQ ID NO: 28622 - protein, 9 aa, synthetic construct
GGEGLDFLT

SEQ ID NO: 28623 - protein, 9 aa, synthetic construct
GGEGADTYY

SEQ ID NO: 28624 - protein, 9 aa, synthetic construct
GGEGNDTVK

SEQ ID NO: 28625 - protein, 9 aa, synthetic construct
GGEGGDLFI

SEQ ID NO: 28626 - protein, 9 aa, synthetic construct
GGEGEDTVI

SEQ ID NO: 28627 - protein, 9 aa, synthetic construct
GGEGKDNLY

SEQ ID NO: 28628 - protein, 9 aa, synthetic construct
GGEGEDQLF

SEQ ID NO: 28629 - protein, 9 aa, synthetic construct
GGEGLDFAI

SEQ ID NO: 28630 - protein, 9 aa, synthetic construct
GGEGHDFIN

SEQ ID NO: 28631 - protein, 9 aa, synthetic construct
GGEGLDELF

SEQ ID NO: 28632 - protein, 9 aa, synthetic construct
GGEGKDQFY

SEQ ID NO: 28633 - protein, 9 aa, synthetic construct
GGEGHDELY

SEQ ID NO: 28634 - protein, 9 aa, synthetic construct
GGEGNDTVH

SEQ ID NO: 28635 - protein, 9 aa, synthetic construct
GGEGADNIA

SEQ ID NO: 28636 - protein, 9 aa, synthetic construct
GGEGNDTVQ

SEQ ID NO: 28637 - protein, 9 aa, synthetic construct
GGEGDDEAH

SEQ ID NO: 28638 - protein, 9 aa, synthetic construct
GGEGKDMLY

SEQ ID NO: 28639 - protein, 9 aa, synthetic construct
GGEGKDMLN

SEQ ID NO: 28640 - protein, 9 aa, synthetic construct
GGEGNDTVS

SEQ ID NO: 28641 - protein, 9 aa, synthetic construct
GGEGDDVIQ

SEQ ID NO: 28642 - protein, 9 aa, synthetic construct
GGEGHDFLF

SEQ ID NO: 28643 - protein, 9 aa, synthetic construct
GGEGDDVIL

SEQ ID NO: 28644 - protein, 9 aa, synthetic construct
GGEGKDMLI

SEQ ID NO: 28645 - protein, 9 aa, synthetic construct
GGEGHDFLI

SEQ ID NO: 28646 - protein, 9 aa, synthetic construct
GGEGKDMLD

SEQ ID NO: 28647 - protein, 9 aa, synthetic construct
GGEGHDFVS

SEQ ID NO: 28648 - protein, 9 aa, synthetic construct
GGEGHDHFV

SEQ ID NO: 28649 - protein, 9 aa, synthetic construct
GGEGADTYI

SEQ ID NO: 28650 - protein, 9 aa, synthetic construct
GGEGNDNAW

SEQ ID NO: 28651 - protein, 9 aa, synthetic construct
GGEGHDHLD

SEQ ID NO: 28652 - protein, 9 aa, synthetic construct
GGEGEDVFA

SEQ ID NO: 28653 - protein, 9 aa, synthetic construct
GGEGADMLK

SEQ ID NO: 28654 - protein, 9 aa, synthetic construct
GGEGDDLMA

SEQ ID NO: 28655 - protein, 9 aa, synthetic construct
GGEGNDLVF

SEQ ID NO: 28656 - protein, 9 aa, synthetic construct
GGEGEDLLQ

SEQ ID NO: 28657 - protein, 9 aa, synthetic construct
GGEGDDLVT

SEQ ID NO: 28658 - protein, 9 aa, synthetic construct
GGEGADLVM

SEQ ID NO: 28659 - protein, 9 aa, synthetic construct
GGEGLDQLY

SEQ ID NO: 28660 - protein, 9 aa, synthetic construct
GGEGADVMD

SEQ ID NO: 28661 - protein, 9 aa, synthetic construct
GGEGADLVR

SEQ ID NO: 28662 - protein, 9 aa, synthetic construct
GGEGADLVS

SEQ ID NO: 28663 - protein, 9 aa, synthetic construct
GGEGDDLVK

SEQ ID NO: 28664 - protein, 9 aa, synthetic construct
GGEGADLVT

SEQ ID NO: 28665 - protein, 9 aa, synthetic construct
GGEGNDTAW

SEQ ID NO: 28666 - protein, 9 aa, synthetic construct
GGEGNDVIQ

SEQ ID NO: 28667 - protein, 9 aa, synthetic construct
GGEGKDKLT

SEQ ID NO: 28668 - protein, 9 aa, synthetic construct
GGEGDDVFI

SEQ ID NO: 28669 - protein, 9 aa, synthetic construct
GGEGDDLVQ

SEQ ID NO: 28670 - protein, 9 aa, synthetic construct
GGEGLDRMF

SEQ ID NO: 28671 - protein, 9 aa, synthetic construct
GGEGNDLVD

SEQ ID NO: 28672 - protein, 9 aa, synthetic construct
GGEGLDRVE

SEQ ID NO: 28673 - protein, 9 aa, synthetic construct
GGEGNDRLG

SEQ ID NO: 28674 - protein, 9 aa, synthetic construct
GGEGADVME

SEQ ID NO: 28675 - protein, 9 aa, synthetic construct
GGEGDDLVY

SEQ ID NO: 28676 - protein, 9 aa, synthetic construct
GGEGDDVFA

SEQ ID NO: 28677 - protein, 9 aa, synthetic construct
GGEGNDFIK

SEQ ID NO: 28678 - protein, 9 aa, synthetic construct
GGEGDDTYS

SEQ ID NO: 28679 - protein, 9 aa, synthetic construct
GGEGDDEIG

SEQ ID NO: 28680 - protein, 9 aa, synthetic construct
GGEGDDYLR

SEQ ID NO: 28681 - protein, 9 aa, synthetic construct
GGEGEDVIV

SEQ ID NO: 28682 - protein, 9 aa, synthetic construct
GGEGADTVQ

SEQ ID NO: 28683 - protein, 9 aa, synthetic construct
GGEGEDVLE

SEQ ID NO: 28684 - protein, 9 aa, synthetic construct
GGEGNDLMS

SEQ ID NO: 28685 - protein, 9 aa, synthetic construct
GGEGNDVLG

SEQ ID NO: 28686 - protein, 9 aa, synthetic construct
GGEGDDIFI

SEQ ID NO: 28687 - protein, 9 aa, synthetic construct
GGEGDDLVN

SEQ ID NO: 28688 - protein, 9 aa, synthetic construct
GGEGNDTAY

SEQ ID NO: 28689 - protein, 9 aa, synthetic construct
GGEGADTVW

SEQ ID NO: 28690 - protein, 9 aa, synthetic construct
GGEGDDYLI

SEQ ID NO: 28691 - protein, 9 aa, synthetic construct
GGEGNDLVL

SEQ ID NO: 28692 - protein, 9 aa, synthetic construct
GGEGDDAFV

SEQ ID NO: 28693 - protein, 9 aa, synthetic construct
GGEGLDLVD

SEQ ID NO: 28694 - protein, 9 aa, synthetic construct
GGEGDDIFR

SEQ ID NO: 28695 - protein, 9 aa, synthetic construct
GGEGDDLMG

SEQ ID NO: 28696 - protein, 9 aa, synthetic construct
GGEGDDLME

SEQ ID NO: 28697 - protein, 9 aa, synthetic construct
GGEGDDEIF

SEQ ID NO: 28698 - protein, 9 aa, synthetic construct
GGEGKDKVA

SEQ ID NO: 28699 - protein, 9 aa, synthetic construct
GGEGADMLF

SEQ ID NO: 28700 - protein, 9 aa, synthetic construct
GGEGNDVAY

SEQ ID NO: 28701 - protein, 9 aa, synthetic construct
GGEGDDAFY

SEQ ID NO: 28702 - protein, 9 aa, synthetic construct
GGEGLDLMY

SEQ ID NO: 28703 - protein, 9 aa, synthetic construct
GGEGNDLVW

SEQ ID NO: 28704 - protein, 9 aa, synthetic construct
GGEGLDLLT

SEQ ID NO: 28705 - protein, 9 aa, synthetic construct
GGEGKDLLD

SEQ ID NO: 28706 - protein, 9 aa, synthetic construct
GGEGADMIL

SEQ ID NO: 28707 - protein, 9 aa, synthetic construct
GGEGGDKMS

SEQ ID NO: 28708 - protein, 9 aa, synthetic construct
GGEGNDVFE

SEQ ID NO: 28709 - protein, 9 aa, synthetic construct
GGEGHDILN

SEQ ID NO: 28710 - protein, 9 aa, synthetic construct
GGEGKDLIY

SEQ ID NO: 28711 - protein, 9 aa, synthetic construct
GGEGLDPVF

SEQ ID NO: 28712 - protein, 9 aa, synthetic construct
GGEGKDKVS

SEQ ID NO: 28713 - protein, 9 aa, synthetic construct
GGEGHDIVR

SEQ ID NO: 28714 - protein, 9 aa, synthetic construct
GGEGADVLW

SEQ ID NO: 28715 - protein, 9 aa, synthetic construct
GGEGEDLLV

SEQ ID NO: 28716 - protein, 9 aa, synthetic construct
GGEGDDLMV

SEQ ID NO: 28717 - protein, 9 aa, synthetic construct
GGEGHDKLD

SEQ ID NO: 28718 - protein, 9 aa, synthetic construct
GGEGDDIFQ

SEQ ID NO: 28719 - protein, 9 aa, synthetic construct
GGEGDDLVD

SEQ ID NO: 28720 - protein, 9 aa, synthetic construct
GGEGNDEYY

SEQ ID NO: 28721 - protein, 9 aa, synthetic construct
GGEGLDQLN

SEQ ID NO: 28722 - protein, 9 aa, synthetic construct
GGEGGDKLQ

SEQ ID NO: 28723 - protein, 9 aa, synthetic construct
GGYGYDYLN

SEQ ID NO: 28724 - protein, 9 aa, synthetic construct
GGEGADHIY

SEQ ID NO: 28725 - protein, 9 aa, synthetic construct
GGAGNDMLC

SEQ ID NO: 28726 - protein, 9 aa, synthetic construct
GGAGNDMFW

SEQ ID NO: 28727 - protein, 9 aa, synthetic construct
GGAGNDMIA

SEQ ID NO: 28728 - protein, 9 aa, synthetic construct
GGAGNDMIE

SEQ ID NO: 28729 - protein, 9 aa, synthetic construct
GGAGNDMII

SEQ ID NO: 28730 - protein, 9 aa, synthetic construct
GGAGNDMIL

SEQ ID NO: 28731 - protein, 9 aa, synthetic construct
GGAGNDMIM

SEQ ID NO: 28732 - protein, 9 aa, synthetic construct
GGAGNDMIN

SEQ ID NO: 28733 - protein, 9 aa, synthetic construct
GGAGNDMIV

SEQ ID NO: 28734 - protein, 9 aa, synthetic construct
GGAGNDMLG

SEQ ID NO: 28735 - protein, 9 aa, synthetic construct
GGAGNDRFS

SEQ ID NO: 28736 - protein, 9 aa, synthetic construct
GGAGNDMLH

SEQ ID NO: 28737 - protein, 9 aa, synthetic construct
GGAGNDMLW

SEQ ID NO: 28738 - protein, 9 aa, synthetic construct
GGAGNDMMA

SEQ ID NO: 28739 - protein, 9 aa, synthetic construct
GGAGNDMMG

SEQ ID NO: 28740 - protein, 9 aa, synthetic construct
GGAGNDMML

SEQ ID NO: 28741 - protein, 9 aa, synthetic construct
GGAGNDMMT

SEQ ID NO: 28742 - protein, 9 aa, synthetic construct
GGAGNDMMY

SEQ ID NO: 28743 - protein, 9 aa, synthetic construct
GGAGNDMVA

SEQ ID NO: 28744 - protein, 9 aa, synthetic construct
GGAGNDMFA

SEQ ID NO: 28745 - protein, 9 aa, synthetic construct
GGAGNDMAH

SEQ ID NO: 28746 - protein, 9 aa, synthetic construct
GGAGNDLYS

SEQ ID NO: 28747 - protein, 9 aa, synthetic construct
GGAGNDLVK

SEQ ID NO: 28748 - protein, 9 aa, synthetic construct
GGAGNDKIQ

SEQ ID NO: 28749 - protein, 9 aa, synthetic construct
GGAGNDKIR

SEQ ID NO: 28750 - protein, 9 aa, synthetic construct
GGAGNDKMH

SEQ ID NO: 28751 - protein, 9 aa, synthetic construct
GGAGNDKMI

SEQ ID NO: 28752 - protein, 9 aa, synthetic construct
GGAGNDKML

SEQ ID NO: 28753 - protein, 9 aa, synthetic construct
GGAGNDKMM

SEQ ID NO: 28754 - protein, 9 aa, synthetic construct
GGAGNDKMR

SEQ ID NO: 28755 - protein, 9 aa, synthetic construct
GGAGNDKMT

SEQ ID NO: 28756 - protein, 9 aa, synthetic construct
GGAGNDKMV

SEQ ID NO: 28757 - protein, 9 aa, synthetic construct
GGAGNDKMW

SEQ ID NO: 28758 - protein, 9 aa, synthetic construct
GGAGNDLAA

SEQ ID NO: 28759 - protein, 9 aa, synthetic construct
GGAGNDLAH

SEQ ID NO: 28760 - protein, 9 aa, synthetic construct
GGAGNDLAI

SEQ ID NO: 28761 - protein, 9 aa, synthetic construct
GGAGNDLAN

SEQ ID NO: 28762 - protein, 9 aa, synthetic construct
GGAGNDLFA

SEQ ID NO: 28763 - protein, 9 aa, synthetic construct
GGAGNDLFS

SEQ ID NO: 28764 - protein, 9 aa, synthetic construct
GGAGNDLMH

SEQ ID NO: 28765 - protein, 9 aa, synthetic construct
GGAGNDMVR

SEQ ID NO: 28766 - protein, 9 aa, synthetic construct
GGAGNDNFG

SEQ ID NO: 28767 - protein, 9 aa, synthetic construct
GGAGNDNIA

SEQ ID NO: 28768 - protein, 9 aa, synthetic construct
GGAGNDQIV

SEQ ID NO: 28769 - protein, 9 aa, synthetic construct
GGAGNDQMK

SEQ ID NO: 28770 - protein, 9 aa, synthetic construct
GGAGNDQMM

SEQ ID NO: 28771 - protein, 9 aa, synthetic construct
GGAGNDQMV

SEQ ID NO: 28772 - protein, 9 aa, synthetic construct
GGAGNDQMY

SEQ ID NO: 28773 - protein, 9 aa, synthetic construct
GGAGNDQVG

SEQ ID NO: 28774 - protein, 9 aa, synthetic construct
GGAGNDQVM

SEQ ID NO: 28775 - protein, 9 aa, synthetic construct
GGAGNDQVR

SEQ ID NO: 28776 - protein, 9 aa, synthetic construct
GGAGNDQYF

SEQ ID NO: 28777 - protein, 9 aa, synthetic construct
GGAGNDQYI

SEQ ID NO: 28778 - protein, 9 aa, synthetic construct
GGAGNDQYR

SEQ ID NO: 28779 - protein, 9 aa, synthetic construct
GGAGNDQYY

SEQ ID NO: 28780 - protein, 9 aa, synthetic construct
GGAGNDRAD

SEQ ID NO: 28781 - protein, 9 aa, synthetic construct
GGAGNDRAS

SEQ ID NO: 28782 - protein, 9 aa, synthetic construct
GGAGNDRAW

SEQ ID NO: 28783 - protein, 9 aa, synthetic construct
GGAGNDRFA

SEQ ID NO: 28784 - protein, 9 aa, synthetic construct
GGAGNDRFH

SEQ ID NO: 28785 - protein, 9 aa, synthetic construct
GGAGNDRFK

SEQ ID NO: 28786 - protein, 9 aa, synthetic construct
GGAGNDQLM

SEQ ID NO: 28787 - protein, 9 aa, synthetic construct
GGAGNDQIM

SEQ ID NO: 28788 - protein, 9 aa, synthetic construct
GGAGNDNIE

SEQ ID NO: 28789 - protein, 9 aa, synthetic construct
GGAGNDQIA

SEQ ID NO: 28790 - protein, 9 aa, synthetic construct
GGAGNDNIH

SEQ ID NO: 28791 - protein, 9 aa, synthetic construct
GGAGNDNII

SEQ ID NO: 28792 - protein, 9 aa, synthetic construct
GGAGNDNIW

SEQ ID NO: 28793 - protein, 9 aa, synthetic construct
GGAGNDNIY

SEQ ID NO: 28794 - protein, 9 aa, synthetic construct
GGAGNDNMG

SEQ ID NO: 28795 - protein, 9 aa, synthetic construct
GGAGNDNMH

SEQ ID NO: 28796 - protein, 9 aa, synthetic construct
GGAGNDNVK

SEQ ID NO: 28797 - protein, 9 aa, synthetic construct
GGAGNDNVT

SEQ ID NO: 28798 - protein, 9 aa, synthetic construct
GGAGNDNYG

SEQ ID NO: 28799 - protein, 9 aa, synthetic construct
GGAGNDNYI

SEQ ID NO: 28800 - protein, 9 aa, synthetic construct
GGAGNDNYL

SEQ ID NO: 28801 - protein, 9 aa, synthetic construct
GGAGNDNYY

SEQ ID NO: 28802 - protein, 9 aa, synthetic construct
GGAGNDQAF

SEQ ID NO: 28803 - protein, 9 aa, synthetic construct
GGAGNDQAQ

SEQ ID NO: 28804 - protein, 9 aa, synthetic construct
GGAGNDQFD

SEQ ID NO: 28805 - protein, 9 aa, synthetic construct
GGAGNDQFF

SEQ ID NO: 28806 - protein, 9 aa, synthetic construct
GGAGNDQFR

SEQ ID NO: 28807 - protein, 9 aa, synthetic construct
GGAGNDKIN

SEQ ID NO: 28808 - protein, 9 aa, synthetic construct
GGAGNDKIK

SEQ ID NO: 28809 - protein, 9 aa, synthetic construct
GGAGNDKIF

SEQ ID NO: 28810 - protein, 9 aa, synthetic construct
GGAGNDEMY

SEQ ID NO: 28811 - protein, 9 aa, synthetic construct
GGAGNDEYV

SEQ ID NO: 28812 - protein, 9 aa, synthetic construct
GGAGNDFAD

SEQ ID NO: 28813 - protein, 9 aa, synthetic construct
GGAGNDFFE

SEQ ID NO: 28814 - protein, 9 aa, synthetic construct
GGAGNDFFG

SEQ ID NO: 28815 - protein, 9 aa, synthetic construct
GGAGNDFFI

SEQ ID NO: 28816 - protein, 9 aa, synthetic construct
GGAGNDFFT

SEQ ID NO: 28817 - protein, 9 aa, synthetic construct
GGAGNDFLW

SEQ ID NO: 28818 - protein, 9 aa, synthetic construct
GGAGNDFME

SEQ ID NO: 28819 - protein, 9 aa, synthetic construct
GGAGNDFMR

SEQ ID NO: 28820 - protein, 9 aa, synthetic construct
GGAGNDFVA

SEQ ID NO: 28821 - protein, 9 aa, synthetic construct
GGAGNDFVF

SEQ ID NO: 28822 - protein, 9 aa, synthetic construct
GGAGNDFVL

SEQ ID NO: 28823 - protein, 9 aa, synthetic construct
GGAGNDFVV

SEQ ID NO: 28824 - protein, 9 aa, synthetic construct
GGAGNDFYD

SEQ ID NO: 28825 - protein, 9 aa, synthetic construct
GGAGNDFYI

SEQ ID NO: 28826 - protein, 9 aa, synthetic construct
GGAGNDFYV

SEQ ID NO: 28827 - protein, 9 aa, synthetic construct
GGAGNDGFQ

SEQ ID NO: 28828 - protein, 9 aa, synthetic construct
GGAGNDEVR

SEQ ID NO: 28829 - protein, 9 aa, synthetic construct
GGAGNDEMR

SEQ ID NO: 28830 - protein, 9 aa, synthetic construct
GGAGNDGID

SEQ ID NO: 28831 - protein, 9 aa, synthetic construct
GGAGNDEMM

SEQ ID NO: 28832 - protein, 9 aa, synthetic construct
GGAGNDDVQ

SEQ ID NO: 28833 - protein, 9 aa, synthetic construct
GGAGNDDVR

SEQ ID NO: 28834 - protein, 9 aa, synthetic construct
GGAGNDDVS

SEQ ID NO: 28835 - protein, 9 aa, synthetic construct
GGAGNDDVT

SEQ ID NO: 28836 - protein, 9 aa, synthetic construct
GGAGNDEAI

SEQ ID NO: 28837 - protein, 9 aa, synthetic construct
GGAGNDEAL

SEQ ID NO: 28838 - protein, 9 aa, synthetic construct
GGAGNDEAR

SEQ ID NO: 28839 - protein, 9 aa, synthetic construct
GGAGNDEFI

SEQ ID NO: 28840 - protein, 9 aa, synthetic construct
GGAGNDEFR

SEQ ID NO: 28841 - protein, 9 aa, synthetic construct
GGAGNDEFT

SEQ ID NO: 28842 - protein, 9 aa, synthetic construct
GGAGNDEFW

SEQ ID NO: 28843 - protein, 9 aa, synthetic construct
GGAGNDEIE

SEQ ID NO: 28844 - protein, 9 aa, synthetic construct
GGAGNDEIF

SEQ ID NO: 28845 - protein, 9 aa, synthetic construct
GGAGNDEIL

SEQ ID NO: 28846 - protein, 9 aa, synthetic construct
GGAGNDEIV

SEQ ID NO: 28847 - protein, 9 aa, synthetic construct
GGAGNDELM

SEQ ID NO: 28848 - protein, 9 aa, synthetic construct
GGAGNDEMD

SEQ ID NO: 28849 - protein, 9 aa, synthetic construct
GGAGNDGFV

SEQ ID NO: 28850 - protein, 9 aa, synthetic construct
GGAGNDGIG

SEQ ID NO: 28851 - protein, 9 aa, synthetic construct
GGAGNDKIA

SEQ ID NO: 28852 - protein, 9 aa, synthetic construct
GGAGNDHYL

SEQ ID NO: 28853 - protein, 9 aa, synthetic construct
GGAGNDIAA

SEQ ID NO: 28854 - protein, 9 aa, synthetic construct
GGAGNDIAE

SEQ ID NO: 28855 - protein, 9 aa, synthetic construct
GGAGNDIAF

SEQ ID NO: 28856 - protein, 9 aa, synthetic construct
GGAGNDIAI

SEQ ID NO: 28857 - protein, 9 aa, synthetic construct
GGAGNDIAN

SEQ ID NO: 28858 - protein, 9 aa, synthetic construct
GGAGNDIFE

SEQ ID NO: 28859 - protein, 9 aa, synthetic construct
GGAGNDIFH

SEQ ID NO: 28860 - protein, 9 aa, synthetic construct
GGAGNDIFS

SEQ ID NO: 28861 - protein, 9 aa, synthetic construct
GGAGNDIIM

SEQ ID NO: 28862 - protein, 9 aa, synthetic construct
GGAGNDIME

SEQ ID NO: 28863 - protein, 9 aa, synthetic construct
GGAGNDIVA

SEQ ID NO: 28864 - protein, 9 aa, synthetic construct
GGAGNDIYG

SEQ ID NO: 28865 - protein, 9 aa, synthetic construct
GGAGNDIYM

SEQ ID NO: 28866 - protein, 9 aa, synthetic construct
GGAGNDIYW

SEQ ID NO: 28867 - protein, 9 aa, synthetic construct
GGAGNDKAY

SEQ ID NO: 28868 - protein, 9 aa, synthetic construct
GGAGNDKFQ

SEQ ID NO: 28869 - protein, 9 aa, synthetic construct
GGAGNDKFS

SEQ ID NO: 28870 - protein, 9 aa, synthetic construct
GGAGNDHYV

SEQ ID NO: 28871 - protein, 9 aa, synthetic construct
GGAGNDHVL

SEQ ID NO: 28872 - protein, 9 aa, synthetic construct
GGAGNDGIH

SEQ ID NO: 28873 - protein, 9 aa, synthetic construct
GGAGNDHMW

SEQ ID NO: 28874 - protein, 9 aa, synthetic construct
GGAGNDGIS

SEQ ID NO: 28875 - protein, 9 aa, synthetic construct
GGAGNDGIY

SEQ ID NO: 28876 - protein, 9 aa, synthetic construct
GGAGNDGLG

SEQ ID NO: 28877 - protein, 9 aa, synthetic construct
GGAGNDGLQ

SEQ ID NO: 28878 - protein, 9 aa, synthetic construct
GGAGNDGVL

SEQ ID NO: 28879 - protein, 9 aa, synthetic construct
GGAGNDGVN

SEQ ID NO: 28880 - protein, 9 aa, synthetic construct
GGAGNDGYL

SEQ ID NO: 28881 - protein, 9 aa, synthetic construct
GGAGNDGYT

SEQ ID NO: 28882 - protein, 9 aa, synthetic construct
GGAGNDHIA

SEQ ID NO: 28883 - protein, 9 aa, synthetic construct
GGAGNDHIG

SEQ ID NO: 28884 - protein, 9 aa, synthetic construct
GGAGNDHIM

SEQ ID NO: 28885 - protein, 9 aa, synthetic construct
GGAGNDHIW

SEQ ID NO: 28886 - protein, 9 aa, synthetic construct
GGAGNDHLG

SEQ ID NO: 28887 - protein, 9 aa, synthetic construct
GGAGNDHLM

SEQ ID NO: 28888 - protein, 9 aa, synthetic construct
GGAGNDHMA

SEQ ID NO: 28889 - protein, 9 aa, synthetic construct
GGAGNDHMN

SEQ ID NO: 28890 - protein, 9 aa, synthetic construct
GGAGNDHMV

SEQ ID NO: 28891 - protein, 9 aa, synthetic construct
GGAGNDRFN

SEQ ID NO: 28892 - protein, 9 aa, synthetic construct
GGAGNDRLX

SEQ ID NO: 28893 - protein, 9 aa, synthetic construct
GGAGNDDVA

SEQ ID NO: 28894 - protein, 9 aa, synthetic construct
GGAGPDRLL

SEQ ID NO: 28895 - protein, 9 aa, synthetic construct
GGAGPDLVD

SEQ ID NO: 28896 - protein, 9 aa, synthetic construct
GGAGPDQLY

SEQ ID NO: 28897 - protein, 9 aa, synthetic construct
GGAGPDQMV

SEQ ID NO: 28898 - protein, 9 aa, synthetic construct
GGAGPDQVW

SEQ ID NO: 28899 - protein, 9 aa, synthetic construct
GGAGPDRFF

SEQ ID NO: 28900 - protein, 9 aa, synthetic construct
GGAGPDRIW

SEQ ID NO: 28901 - protein, 9 aa, synthetic construct
GGAGPDRLF

SEQ ID NO: 28902 - protein, 9 aa, synthetic construct
GGAGPDRLI

SEQ ID NO: 28903 - protein, 9 aa, synthetic construct
GGAGPDRLT

SEQ ID NO: 28904 - protein, 9 aa, synthetic construct
GGAGNDRMG

SEQ ID NO: 28905 - protein, 9 aa, synthetic construct
GGAGPDRME

SEQ ID NO: 28906 - protein, 9 aa, synthetic construct
GGAGPDRMS

SEQ ID NO: 28907 - protein, 9 aa, synthetic construct
GGAGPDSID

SEQ ID NO: 28908 - protein, 9 aa, synthetic construct
GGAGPDSLD

SEQ ID NO: 28909 - protein, 9 aa, synthetic construct
GGAGPDTFE

SEQ ID NO: 28910 - protein, 9 aa, synthetic construct
GGAGPDTIR

SEQ ID NO: 28911 - protein, 9 aa, synthetic construct
GGAGPDTLM

SEQ ID NO: 28912 - protein, 9 aa, synthetic construct
GGAGPDTLV

SEQ ID NO: 28913 - protein, 9 aa, synthetic construct
GGAGPDLLT

SEQ ID NO: 28914 - protein, 9 aa, synthetic construct
GGAGPDLLF

SEQ ID NO: 28915 - protein, 9 aa, synthetic construct
GGAGPDLLD

SEQ ID NO: 28916 - protein, 9 aa, synthetic construct
GGAGPDLFR

SEQ ID NO: 28917 - protein, 9 aa, synthetic construct
GGAGPDAFM

SEQ ID NO: 28918 - protein, 9 aa, synthetic construct
GGAGPDAID

SEQ ID NO: 28919 - protein, 9 aa, synthetic construct
GGAGPDAIE

SEQ ID NO: 28920 - protein, 9 aa, synthetic construct
GGAGPDAML

SEQ ID NO: 28921 - protein, 9 aa, synthetic construct
GGAGPDAVS

SEQ ID NO: 28922 - protein, 9 aa, synthetic construct
GGAGPDELF

SEQ ID NO: 28923 - protein, 9 aa, synthetic construct
GGAGPDGLR

SEQ ID NO: 28924 - protein, 9 aa, synthetic construct
GGAGPDGLW

SEQ ID NO: 28925 - protein, 9 aa, synthetic construct
GGAGPDHFR

SEQ ID NO: 28926 - protein, 9 aa, synthetic construct
GGAGPDHLS

SEQ ID NO: 28927 - protein, 9 aa, synthetic construct
GGAGPDIFV

SEQ ID NO: 28928 - protein, 9 aa, synthetic construct
GGAGPDIIR

SEQ ID NO: 28929 - protein, 9 aa, synthetic construct
GGAGPDILD

SEQ ID NO: 28930 - protein, 9 aa, synthetic construct
GGAGPDILL

SEQ ID NO: 28931 - protein, 9 aa, synthetic construct
GGAGPDIMR

SEQ ID NO: 28932 - protein, 9 aa, synthetic construct
GGAGPDIVK

SEQ ID NO: 28933 - protein, 9 aa, synthetic construct
GGAGPDKFV

SEQ ID NO: 28934 - protein, 9 aa, synthetic construct
GGAGPDTMA

SEQ ID NO: 28935 - protein, 9 aa, synthetic construct
GGAGPDTMK

SEQ ID NO: 28936 - protein, 9 aa, synthetic construct
GGAGPDTMN

SEQ ID NO: 28937 - protein, 9 aa, synthetic construct
GGAGQDDLS

SEQ ID NO: 28938 - protein, 9 aa, synthetic construct
GGAGQDDVK

SEQ ID NO: 28939 - protein, 9 aa, synthetic construct
GGAGQDEIY

SEQ ID NO: 28940 - protein, 9 aa, synthetic construct
GGAGQDELH

SEQ ID NO: 28941 - protein, 9 aa, synthetic construct
GGAGQDELN

SEQ ID NO: 28942 - protein, 9 aa, synthetic construct
GGAGQDELS

SEQ ID NO: 28943 - protein, 9 aa, synthetic construct
GGAGQDEVR

SEQ ID NO: 28944 - protein, 9 aa, synthetic construct
GGAGQDEVV

SEQ ID NO: 28945 - protein, 9 aa, synthetic construct
GGAGQDFAS

SEQ ID NO: 28946 - protein, 9 aa, synthetic construct
GGAGQDFLG

SEQ ID NO: 28947 - protein, 9 aa, synthetic construct
GGAGQDFLN

SEQ ID NO: 28948 - protein, 9 aa, synthetic construct
GGAGQDFLR

SEQ ID NO: 28949 - protein, 9 aa, synthetic construct
GGAGQDFLY

SEQ ID NO: 28950 - protein, 9 aa, synthetic construct
GGAGQDGVF

SEQ ID NO: 28951 - protein, 9 aa, synthetic construct
GGAGQDHLA

SEQ ID NO: 28952 - protein, 9 aa, synthetic construct
GGAGQDHLE

SEQ ID NO: 28953 - protein, 9 aa, synthetic construct
GGAGQDIAV

SEQ ID NO: 28954 - protein, 9 aa, synthetic construct
GGAGQDIFR

SEQ ID NO: 28955 - protein, 9 aa, synthetic construct
GGAGQDDMS

SEQ ID NO: 28956 - protein, 9 aa, synthetic construct
GGAGQDDLR

SEQ ID NO: 28957 - protein, 9 aa, synthetic construct
GGAGPDTMP

SEQ ID NO: 28958 - protein, 9 aa, synthetic construct
GGAGQDDLL

SEQ ID NO: 28959 - protein, 9 aa, synthetic construct
GGAGPDTVQ

SEQ ID NO: 28960 - protein, 9 aa, synthetic construct
GGAGPDTVR

SEQ ID NO: 28961 - protein, 9 aa, synthetic construct
GGAGPDVFV

SEQ ID NO: 28962 - protein, 9 aa, synthetic construct
GGAGPDVID

SEQ ID NO: 28963 - protein, 9 aa, synthetic construct
GGAGPDVLQ

SEQ ID NO: 28964 - protein, 9 aa, synthetic construct
GGAGPDVLS

SEQ ID NO: 28965 - protein, 9 aa, synthetic construct
GGAGPDVLT

SEQ ID NO: 28966 - protein, 9 aa, synthetic construct
GGAGPDVLV

SEQ ID NO: 28967 - protein, 9 aa, synthetic construct
GGAGPDVMS

SEQ ID NO: 28968 - protein, 9 aa, synthetic construct
GGAGPDYLS

SEQ ID NO: 28969 - protein, 9 aa, synthetic construct
GGAGQDAFT

SEQ ID NO: 28970 - protein, 9 aa, synthetic construct
GGAGQDAIE

SEQ ID NO: 28971 - protein, 9 aa, synthetic construct
GGAGQDAIT

SEQ ID NO: 28972 - protein, 9 aa, synthetic construct
GGAGQDALA

SEQ ID NO: 28973 - protein, 9 aa, synthetic construct
GGAGQDALT

SEQ ID NO: 28974 - protein, 9 aa, synthetic construct
GGAGQDAMS

SEQ ID NO: 28975 - protein, 9 aa, synthetic construct
GGAGQDDLK

SEQ ID NO: 28976 - protein, 9 aa, synthetic construct
GGAGPDAFA

SEQ ID NO: 28977 - protein, 9 aa, synthetic construct
GGAGNDYYV

SEQ ID NO: 28978 - protein, 9 aa, synthetic construct
GGAGNDYVV

SEQ ID NO: 28979 - protein, 9 aa, synthetic construct
GGAGNDSIK

SEQ ID NO: 28980 - protein, 9 aa, synthetic construct
GGAGNDSMM

SEQ ID NO: 28981 - protein, 9 aa, synthetic construct
GGAGNDSMN

SEQ ID NO: 28982 - protein, 9 aa, synthetic construct
GGAGNDSVA

SEQ ID NO: 28983 - protein, 9 aa, synthetic construct
GGAGNDSVE

SEQ ID NO: 28984 - protein, 9 aa, synthetic construct
GGAGNDSVI

SEQ ID NO: 28985 - protein, 9 aa, synthetic construct
GGAGNDSVR

SEQ ID NO: 28986 - protein, 9 aa, synthetic construct
GGAGNDSYH

SEQ ID NO: 28987 - protein, 9 aa, synthetic construct
GGAGNDSYK

SEQ ID NO: 28988 - protein, 9 aa, synthetic construct
GGAGNDSYQ

SEQ ID NO: 28989 - protein, 9 aa, synthetic construct
GGAGNDSYS

SEQ ID NO: 28990 - protein, 9 aa, synthetic construct
GGAGNDTAA

SEQ ID NO: 28991 - protein, 9 aa, synthetic construct
GGAGNDTAE

SEQ ID NO: 28992 - protein, 9 aa, synthetic construct
GGAGNDTAG

SEQ ID NO: 28993 - protein, 9 aa, synthetic construct
GGAGNDTAH

SEQ ID NO: 28994 - protein, 9 aa, synthetic construct
GGAGNDTAK

SEQ ID NO: 28995 - protein, 9 aa, synthetic construct
GGAGNDTIC

SEQ ID NO: 28996 - protein, 9 aa, synthetic construct
GGAGNDTLC

SEQ ID NO: 28997 - protein, 9 aa, synthetic construct
GGAGNDSMG

SEQ ID NO: 28998 - protein, 9 aa, synthetic construct
GGAGNDSFT

SEQ ID NO: 28999 - protein, 9 aa, synthetic construct
GGAGNDVAF

SEQ ID NO: 29000 - protein, 9 aa, synthetic construct
GGAGNDSFS

SEQ ID NO: 29001 - protein, 9 aa, synthetic construct
GGAGNDRMQ

SEQ ID NO: 29002 - protein, 9 aa, synthetic construct
GGAGNDRVK

SEQ ID NO: 29003 - protein, 9 aa, synthetic construct
GGAGNDRVT

SEQ ID NO: 29004 - protein, 9 aa, synthetic construct
GGAGNDRVV

SEQ ID NO: 29005 - protein, 9 aa, synthetic construct
GGAGNDRYR

SEQ ID NO: 29006 - protein, 9 aa, synthetic construct
GGAGNDRYY

SEQ ID NO: 29007 - protein, 9 aa, synthetic construct
GGAGNDSAA

SEQ ID NO: 29008 - protein, 9 aa, synthetic construct
GGAGNDSAD

SEQ ID NO: 29009 - protein, 9 aa, synthetic construct
GGAGNDSAG

SEQ ID NO: 29010 - protein, 9 aa, synthetic construct
GGAGNDSAL

SEQ ID NO: 29011 - protein, 9 aa, synthetic construct
GGAGNDSAN

SEQ ID NO: 29012 - protein, 9 aa, synthetic construct
GGAGNDSAT

SEQ ID NO: 29013 - protein, 9 aa, synthetic construct
GGAGNDSFA

SEQ ID NO: 29014 - protein, 9 aa, synthetic construct
GGAGNDSFD

SEQ ID NO: 29015 - protein, 9 aa, synthetic construct
GGAGNDSFE

SEQ ID NO: 29016 - protein, 9 aa, synthetic construct
GGAGNDSFH

SEQ ID NO: 29017 - protein, 9 aa, synthetic construct
GGAGNDSFQ

SEQ ID NO: 29018 - protein, 9 aa, synthetic construct
GGAGNDTMW

SEQ ID NO: 29019 - protein, 9 aa, synthetic construct
GGAGNDVAR

SEQ ID NO: 29020 - protein, 9 aa, synthetic construct
GGAGNDYVI

SEQ ID NO: 29021 - protein, 9 aa, synthetic construct
GGAGNDWIL

SEQ ID NO: 29022 - protein, 9 aa, synthetic construct
GGAGNDWIV

SEQ ID NO: 29023 - protein, 9 aa, synthetic construct
GGAGNDWLM

SEQ ID NO: 29024 - protein, 9 aa, synthetic construct
GGAGNDWMN

SEQ ID NO: 29025 - protein, 9 aa, synthetic construct
GGAGNDWVH

SEQ ID NO: 29026 - protein, 9 aa, synthetic construct
GGAGNDWVN

SEQ ID NO: 29027 - protein, 9 aa, synthetic construct
GGAGNDWVS

SEQ ID NO: 29028 - protein, 9 aa, synthetic construct
GGAGNDWYN

SEQ ID NO: 29029 - protein, 9 aa, synthetic construct
GGAGNDXID

SEQ ID NO: 29030 - protein, 9 aa, synthetic construct
GGAGNDYAF

SEQ ID NO: 29031 - protein, 9 aa, synthetic construct
GGAGNDYAK

SEQ ID NO: 29032 - protein, 9 aa, synthetic construct
GGAGNDYFE

SEQ ID NO: 29033 - protein, 9 aa, synthetic construct
GGAGNDYFR

SEQ ID NO: 29034 - protein, 9 aa, synthetic construct
GGAGNDYFT

SEQ ID NO: 29035 - protein, 9 aa, synthetic construct
GGAGNDYIK

SEQ ID NO: 29036 - protein, 9 aa, synthetic construct
GGAGNDYIR

SEQ ID NO: 29037 - protein, 9 aa, synthetic construct
GGAGNDYMI

SEQ ID NO: 29038 - protein, 9 aa, synthetic construct
GGAGNDYVE

SEQ ID NO: 29039 - protein, 9 aa, synthetic construct
GGAGNDWIT

SEQ ID NO: 29040 - protein, 9 aa, synthetic construct
GGAGNDWIG

SEQ ID NO: 29041 - protein, 9 aa, synthetic construct
GGAGNDVFG

SEQ ID NO: 29042 - protein, 9 aa, synthetic construct
GGAGNDWFR

SEQ ID NO: 29043 - protein, 9 aa, synthetic construct
GGAGNDVFH

SEQ ID NO: 29044 - protein, 9 aa, synthetic construct
GGAGNDVLC

SEQ ID NO: 29045 - protein, 9 aa, synthetic construct
GGAGNDVVE

SEQ ID NO: 29046 - protein, 9 aa, synthetic construct
GGAGNDVVG

SEQ ID NO: 29047 - protein, 9 aa, synthetic construct
GGAGNDVVL

SEQ ID NO: 29048 - protein, 9 aa, synthetic construct
GGAGNDVVM

SEQ ID NO: 29049 - protein, 9 aa, synthetic construct
GGAGNDVVW

SEQ ID NO: 29050 - protein, 9 aa, synthetic construct
GGAGNDVYA

SEQ ID NO: 29051 - protein, 9 aa, synthetic construct
GGAGNDVYD

SEQ ID NO: 29052 - protein, 9 aa, synthetic construct
GGAGNDVYG

SEQ ID NO: 29053 - protein, 9 aa, synthetic construct
GGAGNDVYN

SEQ ID NO: 29054 - protein, 9 aa, synthetic construct
GGAGNDVYS

SEQ ID NO: 29055 - protein, 9 aa, synthetic construct
GGAGNDWAA

SEQ ID NO: 29056 - protein, 9 aa, synthetic construct
GGAGNDWAE

SEQ ID NO: 29057 - protein, 9 aa, synthetic construct
GGAGNDWAR

SEQ ID NO: 29058 - protein, 9 aa, synthetic construct
GGAGNDWAV

SEQ ID NO: 29059 - protein, 9 aa, synthetic construct
GGAGNDWAY

SEQ ID NO: 29060 - protein, 9 aa, synthetic construct
GGAGNDDVL

SEQ ID NO: 29061 - protein, 9 aa, synthetic construct
GGAGNDDMN

SEQ ID NO: 29062 - protein, 9 aa, synthetic construct
GGEGADHFV

SEQ ID NO: 29063 - protein, 9 aa, synthetic construct
GGAGLDDID

SEQ ID NO: 29064 - protein, 9 aa, synthetic construct
GGAGLDALS

SEQ ID NO: 29065 - protein, 9 aa, synthetic construct
GGAGLDALT

SEQ ID NO: 29066 - protein, 9 aa, synthetic construct
GGAGLDAMS

SEQ ID NO: 29067 - protein, 9 aa, synthetic construct
GGAGLDAMY

SEQ ID NO: 29068 - protein, 9 aa, synthetic construct
GGAGLDAVA

SEQ ID NO: 29069 - protein, 9 aa, synthetic construct
GGAGLDAVY

SEQ ID NO: 29070 - protein, 9 aa, synthetic construct
GGAGLDCLS

SEQ ID NO: 29071 - protein, 9 aa, synthetic construct
GGAGLDDFV

SEQ ID NO: 29072 - protein, 9 aa, synthetic construct
GGAGLDDLN

SEQ ID NO: 29073 - protein, 9 aa, synthetic construct
GGAGLDQLF

SEQ ID NO: 29074 - protein, 9 aa, synthetic construct
GGAGLDDLT

SEQ ID NO: 29075 - protein, 9 aa, synthetic construct
GGAGLDEIF

SEQ ID NO: 29076 - protein, 9 aa, synthetic construct
GGAGLDEIT

SEQ ID NO: 29077 - protein, 9 aa, synthetic construct
GGAGLDELF

SEQ ID NO: 29078 - protein, 9 aa, synthetic construct
GGAGLDELI

SEQ ID NO: 29079 - protein, 9 aa, synthetic construct
GGAGLDELV

SEQ ID NO: 29080 - protein, 9 aa, synthetic construct
GGAGLDEMH

SEQ ID NO: 29081 - protein, 9 aa, synthetic construct
GGAGLDEVD

SEQ ID NO: 29082 - protein, 9 aa, synthetic construct
GGAGLDALR

SEQ ID NO: 29083 - protein, 9 aa, synthetic construct
GGAGLDALD

SEQ ID NO: 29084 - protein, 9 aa, synthetic construct
GGAGLDAIS

SEQ ID NO: 29085 - protein, 9 aa, synthetic construct
GGAGKDYVY

SEQ ID NO: 29086 - protein, 9 aa, synthetic construct
GGAGKDVIT

SEQ ID NO: 29087 - protein, 9 aa, synthetic construct
GGAGKDVLF

SEQ ID NO: 29088 - protein, 9 aa, synthetic construct
GGAGKDVLH

SEQ ID NO: 29089 - protein, 9 aa, synthetic construct
GGAGKDVLQ

SEQ ID NO: 29090 - protein, 9 aa, synthetic construct
GGAGKDVMI

SEQ ID NO: 29091 - protein, 9 aa, synthetic construct
GGAGKDVML

SEQ ID NO: 29092 - protein, 9 aa, synthetic construct
GGAGKDVMY

SEQ ID NO: 29093 - protein, 9 aa, synthetic construct
GGAGKDVVN

SEQ ID NO: 29094 - protein, 9 aa, synthetic construct
GGAGKDVVT

SEQ ID NO: 29095 - protein, 9 aa, synthetic construct
GGAGKDWIK

SEQ ID NO: 29096 - protein, 9 aa, synthetic construct
GGAGKDWIR

SEQ ID NO: 29097 - protein, 9 aa, synthetic construct
GGAGKDYAS

SEQ ID NO: 29098 - protein, 9 aa, synthetic construct
GGAGKDYAV

SEQ ID NO: 29099 - protein, 9 aa, synthetic construct
GGAGKDYFV

SEQ ID NO: 29100 - protein, 9 aa, synthetic construct
GGAGKDYLA

SEQ ID NO: 29101 - protein, 9 aa, synthetic construct
GGAGKDYLL

SEQ ID NO: 29102 - protein, 9 aa, synthetic construct
GGAGKDYVS

SEQ ID NO: 29103 - protein, 9 aa, synthetic construct
GGAGLDEVR

SEQ ID NO: 29104 - protein, 9 aa, synthetic construct
GGAGLDFAL

SEQ ID NO: 29105 - protein, 9 aa, synthetic construct
GGAGLDFAT

SEQ ID NO: 29106 - protein, 9 aa, synthetic construct
GGAGLDLAY

SEQ ID NO: 29107 - protein, 9 aa, synthetic construct
GGAGLDLLF

SEQ ID NO: 29108 - protein, 9 aa, synthetic construct
GGAGLDLLH

SEQ ID NO: 29109 - protein, 9 aa, synthetic construct
GGAGLDLLR

SEQ ID NO: 29110 - protein, 9 aa, synthetic construct
GGAGLDLLS

SEQ ID NO: 29111 - protein, 9 aa, synthetic construct
GGAGLDLLV

SEQ ID NO: 29112 - protein, 9 aa, synthetic construct
GGAGLDLMV

SEQ ID NO: 29113 - protein, 9 aa, synthetic construct
GGAGLDLYS

SEQ ID NO: 29114 - protein, 9 aa, synthetic construct
GGAGLDMAD

SEQ ID NO: 29115 - protein, 9 aa, synthetic construct
GGAGLDMLS

SEQ ID NO: 29116 - protein, 9 aa, synthetic construct
GGAGLDNFR

SEQ ID NO: 29117 - protein, 9 aa, synthetic construct
GGAGLDNID

SEQ ID NO: 29118 - protein, 9 aa, synthetic construct
GGAGLDNIL

SEQ ID NO: 29119 - protein, 9 aa, synthetic construct
GGAGLDNLF

SEQ ID NO: 29120 - protein, 9 aa, synthetic construct
GGAGLDNLT

SEQ ID NO: 29121 - protein, 9 aa, synthetic construct
GGAGLDNMN

SEQ ID NO: 29122 - protein, 9 aa, synthetic construct
GGAGLDNMS

SEQ ID NO: 29123 - protein, 9 aa, synthetic construct
GGAGLDQFN

SEQ ID NO: 29124 - protein, 9 aa, synthetic construct
GGAGLDLIF

SEQ ID NO: 29125 - protein, 9 aa, synthetic construct
GGAGLDLAV

SEQ ID NO: 29126 - protein, 9 aa, synthetic construct
GGAGLDFIL

SEQ ID NO: 29127 - protein, 9 aa, synthetic construct
GGAGLDLAS

SEQ ID NO: 29128 - protein, 9 aa, synthetic construct
GGAGLDFLI

SEQ ID NO: 29129 - protein, 9 aa, synthetic construct
GGAGLDGMT

SEQ ID NO: 29130 - protein, 9 aa, synthetic construct
GGAGLDHIW

SEQ ID NO: 29131 - protein, 9 aa, synthetic construct
GGAGLDIAS

SEQ ID NO: 29132 - protein, 9 aa, synthetic construct
GGAGLDIAV

SEQ ID NO: 29133 - protein, 9 aa, synthetic construct
GGAGLDIIE

SEQ ID NO: 29134 - protein, 9 aa, synthetic construct
GGAGLDILA

SEQ ID NO: 29135 - protein, 9 aa, synthetic construct
GGAGLDILD

SEQ ID NO: 29136 - protein, 9 aa, synthetic construct
GGAGLDILE

SEQ ID NO: 29137 - protein, 9 aa, synthetic construct
GGAGLDILS

SEQ ID NO: 29138 - protein, 9 aa, synthetic construct
GGAGLDIMT

SEQ ID NO: 29139 - protein, 9 aa, synthetic construct
GGAGLDIVN

SEQ ID NO: 29140 - protein, 9 aa, synthetic construct
GGAGLDKFI

SEQ ID NO: 29141 - protein, 9 aa, synthetic construct
GGAGLDKIY

SEQ ID NO: 29142 - protein, 9 aa, synthetic construct
GGAGLDKLA

SEQ ID NO: 29143 - protein, 9 aa, synthetic construct
GGAGLDKLF

SEQ ID NO: 29144 - protein, 9 aa, synthetic construct
GGAGLDKMV

SEQ ID NO: 29145 - protein, 9 aa, synthetic construct
GGAGKDVIN

SEQ ID NO: 29146 - protein, 9 aa, synthetic construct
GGAGKDVIE

SEQ ID NO: 29147 - protein, 9 aa, synthetic construct
GGAGKDVID

SEQ ID NO: 29148 - protein, 9 aa, synthetic construct
GGAGKDLLY

SEQ ID NO: 29149 - protein, 9 aa, synthetic construct
GGAGKDLVE

SEQ ID NO: 29150 - protein, 9 aa, synthetic construct
GGAGKDMAD

SEQ ID NO: 29151 - protein, 9 aa, synthetic construct
GGAGKDMAS

SEQ ID NO: 29152 - protein, 9 aa, synthetic construct
GGAGKDMFA

SEQ ID NO: 29153 - protein, 9 aa, synthetic construct
GGAGKDMMD

SEQ ID NO: 29154 - protein, 9 aa, synthetic construct
GGAGKDNLD

SEQ ID NO: 29155 - protein, 9 aa, synthetic construct
GGAGKDNLT

SEQ ID NO: 29156 - protein, 9 aa, synthetic construct
GGAGKDQFL

SEQ ID NO: 29157 - protein, 9 aa, synthetic construct
GGAGKDQIE

SEQ ID NO: 29158 - protein, 9 aa, synthetic construct
GGAGKDQIR

SEQ ID NO: 29159 - protein, 9 aa, synthetic construct
GGAGKDQLA

SEQ ID NO: 29160 - protein, 9 aa, synthetic construct
GGAGKDQLE

SEQ ID NO: 29161 - protein, 9 aa, synthetic construct
GGAGKDQLH

SEQ ID NO: 29162 - protein, 9 aa, synthetic construct
GGAGKDQLL

SEQ ID NO: 29163 - protein, 9 aa, synthetic construct
GGAGKDQLN

SEQ ID NO: 29164 - protein, 9 aa, synthetic construct
GGAGKDQLR

SEQ ID NO: 29165 - protein, 9 aa, synthetic construct
GGAGKDQLS

SEQ ID NO: 29166 - protein, 9 aa, synthetic construct
GGAGKDLMT

SEQ ID NO: 29167 - protein, 9 aa, synthetic construct
GGAGKDLLT

SEQ ID NO: 29168 - protein, 9 aa, synthetic construct
GGAGKDQME

SEQ ID NO: 29169 - protein, 9 aa, synthetic construct
GGAGKDLLQ

SEQ ID NO: 29170 - protein, 9 aa, synthetic construct
GGAGKDIVR

SEQ ID NO: 29171 - protein, 9 aa, synthetic construct
GGAGKDIYV

SEQ ID NO: 29172 - protein, 9 aa, synthetic construct
GGAGKDKFV

SEQ ID NO: 29173 - protein, 9 aa, synthetic construct
GGAGKDKIF

SEQ ID NO: 29174 - protein, 9 aa, synthetic construct
GGAGKDKIN

SEQ ID NO: 29175 - protein, 9 aa, synthetic construct
GGAGKDKIS

SEQ ID NO: 29176 - protein, 9 aa, synthetic construct
GGAGKDKIT

SEQ ID NO: 29177 - protein, 9 aa, synthetic construct
GGAGKDKLH

SEQ ID NO: 29178 - protein, 9 aa, synthetic construct
GGAGKDKLK

SEQ ID NO: 29179 - protein, 9 aa, synthetic construct
GGAGKDKLW

SEQ ID NO: 29180 - protein, 9 aa, synthetic construct
GGAGKDKVF

SEQ ID NO: 29181 - protein, 9 aa, synthetic construct
GGAGKDKVN

SEQ ID NO: 29182 - protein, 9 aa, synthetic construct
GGAGKDLFG

SEQ ID NO: 29183 - protein, 9 aa, synthetic construct
GGAGKDLFR

SEQ ID NO: 29184 - protein, 9 aa, synthetic construct
GGAGKDLIS

SEQ ID NO: 29185 - protein, 9 aa, synthetic construct
GGAGKDLLA

SEQ ID NO: 29186 - protein, 9 aa, synthetic construct
GGAGKDLLE

SEQ ID NO: 29187 - protein, 9 aa, synthetic construct
GGAGKDQLT

SEQ ID NO: 29188 - protein, 9 aa, synthetic construct
GGAGKDQVS

SEQ ID NO: 29189 - protein, 9 aa, synthetic construct
GGAGKDVFT

SEQ ID NO: 29190 - protein, 9 aa, synthetic construct
GGAGKDTFT

SEQ ID NO: 29191 - protein, 9 aa, synthetic construct
GGAGKDTIF

SEQ ID NO: 29192 - protein, 9 aa, synthetic construct
GGAGKDTIG

SEQ ID NO: 29193 - protein, 9 aa, synthetic construct
GGAGKDTII

SEQ ID NO: 29194 - protein, 9 aa, synthetic construct
GGAGKDTIL

SEQ ID NO: 29195 - protein, 9 aa, synthetic construct
GGAGKDTIQ

SEQ ID NO: 29196 - protein, 9 aa, synthetic construct
GGAGKDTLF

SEQ ID NO: 29197 - protein, 9 aa, synthetic construct
GGAGKDTLP

SEQ ID NO: 29198 - protein, 9 aa, synthetic construct
GGAGKDTMK

SEQ ID NO: 29199 - protein, 9 aa, synthetic construct
GGAGKDTML

SEQ ID NO: 29200 - protein, 9 aa, synthetic construct
GGAGKDTMS

SEQ ID NO: 29201 - protein, 9 aa, synthetic construct
GGAGKDTVE

SEQ ID NO: 29202 - protein, 9 aa, synthetic construct
GGAGKDTVL

SEQ ID NO: 29203 - protein, 9 aa, synthetic construct
GGAGKDTYD

SEQ ID NO: 29204 - protein, 9 aa, synthetic construct
GGAGKDTYE

SEQ ID NO: 29205 - protein, 9 aa, synthetic construct
GGAGKDVAY

SEQ ID NO: 29206 - protein, 9 aa, synthetic construct
GGAGKDVFG

SEQ ID NO: 29207 - protein, 9 aa, synthetic construct
GGAGKDVFK

SEQ ID NO: 29208 - protein, 9 aa, synthetic construct
GGAGKDTIE

SEQ ID NO: 29209 - protein, 9 aa, synthetic construct
GGAGKDTFR

SEQ ID NO: 29210 - protein, 9 aa, synthetic construct
GGAGKDRIL

SEQ ID NO: 29211 - protein, 9 aa, synthetic construct
GGAGKDTAR

SEQ ID NO: 29212 - protein, 9 aa, synthetic construct
GGAGKDRIS

SEQ ID NO: 29213 - protein, 9 aa, synthetic construct
GGAGKDRME

SEQ ID NO: 29214 - protein, 9 aa, synthetic construct
GGAGKDRMF

SEQ ID NO: 29215 - protein, 9 aa, synthetic construct
GGAGKDRMS

SEQ ID NO: 29216 - protein, 9 aa, synthetic construct
GGAGKDRMT

SEQ ID NO: 29217 - protein, 9 aa, synthetic construct
GGAGKDRMY

SEQ ID NO: 29218 - protein, 9 aa, synthetic construct
GGAGKDRYE

SEQ ID NO: 29219 - protein, 9 aa, synthetic construct
GGAGKDSAL

SEQ ID NO: 29220 - protein, 9 aa, synthetic construct
GGAGKDSFY

SEQ ID NO: 29221 - protein, 9 aa, synthetic construct
GGAGKDSIQ

SEQ ID NO: 29222 - protein, 9 aa, synthetic construct
GGAGKDSLL

SEQ ID NO: 29223 - protein, 9 aa, synthetic construct
GGAGKDSLR

SEQ ID NO: 29224 - protein, 9 aa, synthetic construct
GGAGKDSMS

SEQ ID NO: 29225 - protein, 9 aa, synthetic construct
GGAGKDSVS

SEQ ID NO: 29226 - protein, 9 aa, synthetic construct
GGAGKDSVT

SEQ ID NO: 29227 - protein, 9 aa, synthetic construct
GGAGKDSVY

SEQ ID NO: 29228 - protein, 9 aa, synthetic construct
GGAGKDTAD

SEQ ID NO: 29229 - protein, 9 aa, synthetic construct
GGAGLDQFW

SEQ ID NO: 29230 - protein, 9 aa, synthetic construct
GGAGLDQLK

SEQ ID NO: 29231 - protein, 9 aa, synthetic construct
GGAGNDDMH

SEQ ID NO: 29232 - protein, 9 aa, synthetic construct
GGAGMDSLQ

SEQ ID NO: 29233 - protein, 9 aa, synthetic construct
GGAGMDRLV

SEQ ID NO: 29234 - protein, 9 aa, synthetic construct
GGAGMDRME

SEQ ID NO: 29235 - protein, 9 aa, synthetic construct
GGAGMDSIH

SEQ ID NO: 29236 - protein, 9 aa, synthetic construct
GGAGMDSIQ

SEQ ID NO: 29237 - protein, 9 aa, synthetic construct
GGAGMDSIT

SEQ ID NO: 29238 - protein, 9 aa, synthetic construct
GGAGMDSLD

SEQ ID NO: 29239 - protein, 9 aa, synthetic construct
GGAGMDSLH

SEQ ID NO: 29240 - protein, 9 aa, synthetic construct
GGAGMDSLK

SEQ ID NO: 29241 - protein, 9 aa, synthetic construct
GGAGMDTAD

SEQ ID NO: 29242 - protein, 9 aa, synthetic construct
GGAGLDQLR

SEQ ID NO: 29243 - protein, 9 aa, synthetic construct
GGAGMDTAF

SEQ ID NO: 29244 - protein, 9 aa, synthetic construct
GGAGMDTAQ

SEQ ID NO: 29245 - protein, 9 aa, synthetic construct
GGAGMDTFY

SEQ ID NO: 29246 - protein, 9 aa, synthetic construct
GGAGMDTIE

SEQ ID NO: 29247 - protein, 9 aa, synthetic construct
GGAGMDTIM

SEQ ID NO: 29248 - protein, 9 aa, synthetic construct
GGAGMDTIS

SEQ ID NO: 29249 - protein, 9 aa, synthetic construct
GGAGMDTIV

SEQ ID NO: 29250 - protein, 9 aa, synthetic construct
GGAGMDTLE

SEQ ID NO: 29251 - protein, 9 aa, synthetic construct
GGAGMDRLN

SEQ ID NO: 29252 - protein, 9 aa, synthetic construct
GGAGMDRLM

SEQ ID NO: 29253 - protein, 9 aa, synthetic construct
GGAGMDRID

SEQ ID NO: 29254 - protein, 9 aa, synthetic construct
GGAGMDRFV

SEQ ID NO: 29255 - protein, 9 aa, synthetic construct
GGAGMDFLD

SEQ ID NO: 29256 - protein, 9 aa, synthetic construct
GGAGMDHLS

SEQ ID NO: 29257 - protein, 9 aa, synthetic construct
GGAGMDILE

SEQ ID NO: 29258 - protein, 9 aa, synthetic construct
GGAGMDILI

SEQ ID NO: 29259 - protein, 9 aa, synthetic construct
GGAGMDILQ

SEQ ID NO: 29260 - protein, 9 aa, synthetic construct
GGAGMDIMI

SEQ ID NO: 29261 - protein, 9 aa, synthetic construct
GGAGMDKIY

SEQ ID NO: 29262 - protein, 9 aa, synthetic construct
GGAGMDKLH

SEQ ID NO: 29263 - protein, 9 aa, synthetic construct
GGAGMDKLV

SEQ ID NO: 29264 - protein, 9 aa, synthetic construct
GGAGMDLFH

SEQ ID NO: 29265 - protein, 9 aa, synthetic construct
GGAGMDLFV

SEQ ID NO: 29266 - protein, 9 aa, synthetic construct
GGAGMDLLS

SEQ ID NO: 29267 - protein, 9 aa, synthetic construct
GGAGMDMLI

SEQ ID NO: 29268 - protein, 9 aa, synthetic construct
GGAGMDMLS

SEQ ID NO: 29269 - protein, 9 aa, synthetic construct
GGAGMDNIS

SEQ ID NO: 29270 - protein, 9 aa, synthetic construct
GGAGMDQLG

SEQ ID NO: 29271 - protein, 9 aa, synthetic construct
GGAGMDRFD

SEQ ID NO: 29272 - protein, 9 aa, synthetic construct
GGAGMDTLH

SEQ ID NO: 29273 - protein, 9 aa, synthetic construct
GGAGMDTLR

SEQ ID NO: 29274 - protein, 9 aa, synthetic construct
GGAGMDTMT

SEQ ID NO: 29275 - protein, 9 aa, synthetic construct
GGAGNDAYS

SEQ ID NO: 29276 - protein, 9 aa, synthetic construct
GGAGNDCIM

SEQ ID NO: 29277 - protein, 9 aa, synthetic construct
GGAGNDCIN

SEQ ID NO: 29278 - protein, 9 aa, synthetic construct
GGAGNDCIY

SEQ ID NO: 29279 - protein, 9 aa, synthetic construct
GGAGNDCLD

SEQ ID NO: 29280 - protein, 9 aa, synthetic construct
GGAGNDCLN

SEQ ID NO: 29281 - protein, 9 aa, synthetic construct
GGAGNDCLY

SEQ ID NO: 29282 - protein, 9 aa, synthetic construct
GGAGNDDAT

SEQ ID NO: 29283 - protein, 9 aa, synthetic construct
GGAGNDDFF

SEQ ID NO: 29284 - protein, 9 aa, synthetic construct
GGAGNDDIF

SEQ ID NO: 29285 - protein, 9 aa, synthetic construct
GGAGNDDII

SEQ ID NO: 29286 - protein, 9 aa, synthetic construct
GGAGNDDIK

SEQ ID NO: 29287 - protein, 9 aa, synthetic construct
GGAGNDDIR

SEQ ID NO: 29288 - protein, 9 aa, synthetic construct
GGAGNDDLI

SEQ ID NO: 29289 - protein, 9 aa, synthetic construct
GGAGNDDLK

SEQ ID NO: 29290 - protein, 9 aa, synthetic construct
GGAGNDDMA

SEQ ID NO: 29291 - protein, 9 aa, synthetic construct
GGAGNDDMD

SEQ ID NO: 29292 - protein, 9 aa, synthetic construct
GGAGNDDME

SEQ ID NO: 29293 - protein, 9 aa, synthetic construct
GGAGNDCIA

SEQ ID NO: 29294 - protein, 9 aa, synthetic construct
GGAGNDAYR

SEQ ID NO: 29295 - protein, 9 aa, synthetic construct
GGAGMDVAS

SEQ ID NO: 29296 - protein, 9 aa, synthetic construct
GGAGNDAYF

SEQ ID NO: 29297 - protein, 9 aa, synthetic construct
GGAGMDVFK

SEQ ID NO: 29298 - protein, 9 aa, synthetic construct
GGAGMDVIA

SEQ ID NO: 29299 - protein, 9 aa, synthetic construct
GGAGMDVIF

SEQ ID NO: 29300 - protein, 9 aa, synthetic construct
GGAGMDVIS

SEQ ID NO: 29301 - protein, 9 aa, synthetic construct
GGAGMDVLD

SEQ ID NO: 29302 - protein, 9 aa, synthetic construct
GGAGMDVLS

SEQ ID NO: 29303 - protein, 9 aa, synthetic construct
GGAGMDVMN

SEQ ID NO: 29304 - protein, 9 aa, synthetic construct
GGAGMDWLF

SEQ ID NO: 29305 - protein, 9 aa, synthetic construct
GGAGMDYLE

SEQ ID NO: 29306 - protein, 9 aa, synthetic construct
GGAGNDAAW

SEQ ID NO: 29307 - protein, 9 aa, synthetic construct
GGAGNDAFT

SEQ ID NO: 29308 - protein, 9 aa, synthetic construct
GGAGNDAIR

SEQ ID NO: 29309 - protein, 9 aa, synthetic construct
GGAGNDALC

SEQ ID NO: 29310 - protein, 9 aa, synthetic construct
GGAGNDAMR

SEQ ID NO: 29311 - protein, 9 aa, synthetic construct
GGAGNDAMW

SEQ ID NO: 29312 - protein, 9 aa, synthetic construct
GGAGNDAVD

SEQ ID NO: 29313 - protein, 9 aa, synthetic construct
GGAGNDAVI

SEQ ID NO: 29314 - protein, 9 aa, synthetic construct
GGAGMDFID

SEQ ID NO: 29315 - protein, 9 aa, synthetic construct
GGAGMDFAD

SEQ ID NO: 29316 - protein, 9 aa, synthetic construct
GGAGMDDLH

SEQ ID NO: 29317 - protein, 9 aa, synthetic construct
GGAGLDSLS

SEQ ID NO: 29318 - protein, 9 aa, synthetic construct
GGAGLDTAA

SEQ ID NO: 29319 - protein, 9 aa, synthetic construct
GGAGLDTAF

SEQ ID NO: 29320 - protein, 9 aa, synthetic construct
GGAGLDTAG

SEQ ID NO: 29321 - protein, 9 aa, synthetic construct
GGAGLDTAL

SEQ ID NO: 29322 - protein, 9 aa, synthetic construct
GGAGLDTAQ

SEQ ID NO: 29323 - protein, 9 aa, synthetic construct
GGAGLDTFQ

SEQ ID NO: 29324 - protein, 9 aa, synthetic construct
GGAGLDTFT

SEQ ID NO: 29325 - protein, 9 aa, synthetic construct
GGAGLDTIN

SEQ ID NO: 29326 - protein, 9 aa, synthetic construct
GGAGLDTIQ

SEQ ID NO: 29327 - protein, 9 aa, synthetic construct
GGAGLDTIR

SEQ ID NO: 29328 - protein, 9 aa, synthetic construct
GGAGLDTIT

SEQ ID NO: 29329 - protein, 9 aa, synthetic construct
GGAGLDTIV

SEQ ID NO: 29330 - protein, 9 aa, synthetic construct
GGAGLDTIW

SEQ ID NO: 29331 - protein, 9 aa, synthetic construct
GGAGLDTLH

SEQ ID NO: 29332 - protein, 9 aa, synthetic construct
GGAGLDTLQ

SEQ ID NO: 29333 - protein, 9 aa, synthetic construct
GGAGLDTLR

SEQ ID NO: 29334 - protein, 9 aa, synthetic construct
GGAGLDTLW

SEQ ID NO: 29335 - protein, 9 aa, synthetic construct
GGAGLDSMA

SEQ ID NO: 29336 - protein, 9 aa, synthetic construct
GGAGLDSLL

SEQ ID NO: 29337 - protein, 9 aa, synthetic construct
GGAGLDTMG

SEQ ID NO: 29338 - protein, 9 aa, synthetic construct
GGAGLDSLF

SEQ ID NO: 29339 - protein, 9 aa, synthetic construct
GGAGLDQLT

SEQ ID NO: 29340 - protein, 9 aa, synthetic construct
GGAGLDRFT

SEQ ID NO: 29341 - protein, 9 aa, synthetic construct
GGAGLDRFV

SEQ ID NO: 29342 - protein, 9 aa, synthetic construct
GGAGLDRLH

SEQ ID NO: 29343 - protein, 9 aa, synthetic construct
GGAGLDRLI

SEQ ID NO: 29344 - protein, 9 aa, synthetic construct
GGAGLDRMY

SEQ ID NO: 29345 - protein, 9 aa, synthetic construct
GGAGLDRVF

SEQ ID NO: 29346 - protein, 9 aa, synthetic construct
GGAGLDRVN

SEQ ID NO: 29347 - protein, 9 aa, synthetic construct
GGAGLDRYD

SEQ ID NO: 29348 - protein, 9 aa, synthetic construct
GGAGLDSAR

SEQ ID NO: 29349 - protein, 9 aa, synthetic construct
GGAGLDSFD

SEQ ID NO: 29350 - protein, 9 aa, synthetic construct
GGAGLDSFR

SEQ ID NO: 29351 - protein, 9 aa, synthetic construct
GGAGLDSFS

SEQ ID NO: 29352 - protein, 9 aa, synthetic construct
GGAGLDSIK

SEQ ID NO: 29353 - protein, 9 aa, synthetic construct
GGAGLDSIR

SEQ ID NO: 29354 - protein, 9 aa, synthetic construct
GGAGLDSLA

SEQ ID NO: 29355 - protein, 9 aa, synthetic construct
GGAGLDSLD

SEQ ID NO: 29356 - protein, 9 aa, synthetic construct
GGAGLDTMF

SEQ ID NO: 29357 - protein, 9 aa, synthetic construct
GGAGLDTML

SEQ ID NO: 29358 - protein, 9 aa, synthetic construct
GGAGMDDIQ

SEQ ID NO: 29359 - protein, 9 aa, synthetic construct
GGAGLDVLE

SEQ ID NO: 29360 - protein, 9 aa, synthetic construct
GGAGLDVMA

SEQ ID NO: 29361 - protein, 9 aa, synthetic construct
GGAGLDVMN

SEQ ID NO: 29362 - protein, 9 aa, synthetic construct
GGAGLDVMV

SEQ ID NO: 29363 - protein, 9 aa, synthetic construct
GGAGLDVYF

SEQ ID NO: 29364 - protein, 9 aa, synthetic construct
GGAGLDWAS

SEQ ID NO: 29365 - protein, 9 aa, synthetic construct
GGAGLDWLD

SEQ ID NO: 29366 - protein, 9 aa, synthetic construct
GGAGLDWLR

SEQ ID NO: 29367 - protein, 9 aa, synthetic construct
GGAGLDWLS

SEQ ID NO: 29368 - protein, 9 aa, synthetic construct
GGAGLDWLV

SEQ ID NO: 29369 - protein, 9 aa, synthetic construct
GGAGLDWLW

SEQ ID NO: 29370 - protein, 9 aa, synthetic construct
GGAGLDWVR

SEQ ID NO: 29371 - protein, 9 aa, synthetic construct
GGAGLDYFL

SEQ ID NO: 29372 - protein, 9 aa, synthetic construct
GGAGLDYFS

SEQ ID NO: 29373 - protein, 9 aa, synthetic construct
GGAGLDYID

SEQ ID NO: 29374 - protein, 9 aa, synthetic construct
GGAGLDYLR

SEQ ID NO: 29375 - protein, 9 aa, synthetic construct
GGAGLDYMY

SEQ ID NO: 29376 - protein, 9 aa, synthetic construct
GGAGMDAVD

SEQ ID NO: 29377 - protein, 9 aa, synthetic construct
GGAGLDVLF

SEQ ID NO: 29378 - protein, 9 aa, synthetic construct
GGAGLDVIV

SEQ ID NO: 29379 - protein, 9 aa, synthetic construct
GGAGLDTMQ

SEQ ID NO: 29380 - protein, 9 aa, synthetic construct
GGAGLDVIT

SEQ ID NO: 29381 - protein, 9 aa, synthetic construct
GGAGLDTMV

SEQ ID NO: 29382 - protein, 9 aa, synthetic construct
GGAGLDTMY

SEQ ID NO: 29383 - protein, 9 aa, synthetic construct
GGAGLDTVM

SEQ ID NO: 29384 - protein, 9 aa, synthetic construct
GGAGLDTVS

SEQ ID NO: 29385 - protein, 9 aa, synthetic construct
GGAGLDTVV

SEQ ID NO: 29386 - protein, 9 aa, synthetic construct
GGAGLDTYI

SEQ ID NO: 29387 - protein, 9 aa, synthetic construct
GGAGLDVAD

SEQ ID NO: 29388 - protein, 9 aa, synthetic construct
GGAGLDVAR

SEQ ID NO: 29389 - protein, 9 aa, synthetic construct
GGAGLDVAT

SEQ ID NO: 29390 - protein, 9 aa, synthetic construct
GGAGLDVAV

SEQ ID NO: 29391 - protein, 9 aa, synthetic construct
GGAGLDVFI

SEQ ID NO: 29392 - protein, 9 aa, synthetic construct
GGAGLDVFR

SEQ ID NO: 29393 - protein, 9 aa, synthetic construct
GGAGLDVFT

SEQ ID NO: 29394 - protein, 9 aa, synthetic construct
GGAGLDVFV

SEQ ID NO: 29395 - protein, 9 aa, synthetic construct
GGAGLDVID

SEQ ID NO: 29396 - protein, 9 aa, synthetic construct
GGAGLDVIR

SEQ ID NO: 29397 - protein, 9 aa, synthetic construct
GGAGLDVIS

SEQ ID NO: 29398 - protein, 9 aa, synthetic construct
GGAGQDILE

SEQ ID NO: 29399 - protein, 9 aa, synthetic construct
GGAGQDILF

SEQ ID NO: 29400 - protein, 9 aa, synthetic construct
GGAGQDILI

SEQ ID NO: 29401 - protein, 9 aa, synthetic construct
GGAGSDMLA

SEQ ID NO: 29402 - protein, 9 aa, synthetic construct
GGAGSDLVN

SEQ ID NO: 29403 - protein, 9 aa, synthetic construct
GGAGSDLVS

SEQ ID NO: 29404 - protein, 9 aa, synthetic construct
GGAGSDLVV

SEQ ID NO: 29405 - protein, 9 aa, synthetic construct
GGAGSDLYE

SEQ ID NO: 29406 - protein, 9 aa, synthetic construct
GGAGSDMAD

SEQ ID NO: 29407 - protein, 9 aa, synthetic construct
GGAGSDMIH

SEQ ID NO: 29408 - protein, 9 aa, synthetic construct
GGAGSDMII

SEQ ID NO: 29409 - protein, 9 aa, synthetic construct
GGAGSDMIW

SEQ ID NO: 29410 - protein, 9 aa, synthetic construct
GGAGSDMLT

SEQ ID NO: 29411 - protein, 9 aa, synthetic construct
GGAGSDSLG

SEQ ID NO: 29412 - protein, 9 aa, synthetic construct
GGAGSDMLV

SEQ ID NO: 29413 - protein, 9 aa, synthetic construct
GGAGSDNIA

SEQ ID NO: 29414 - protein, 9 aa, synthetic construct
GGAGSDNIF

SEQ ID NO: 29415 - protein, 9 aa, synthetic construct
GGAGSDNIG

SEQ ID NO: 29416 - protein, 9 aa, synthetic construct
GGAGSDNIS

SEQ ID NO: 29417 - protein, 9 aa, synthetic construct
GGAGSDNIT

SEQ ID NO: 29418 - protein, 9 aa, synthetic construct
GGAGSDNLA

SEQ ID NO: 29419 - protein, 9 aa, synthetic construct
GGAGSDNLE

SEQ ID NO: 29420 - protein, 9 aa, synthetic construct
GGAGSDLVH

SEQ ID NO: 29421 - protein, 9 aa, synthetic construct
GGAGSDLVD

SEQ ID NO: 29422 - protein, 9 aa, synthetic construct
GGAGSDLMY

SEQ ID NO: 29423 - protein, 9 aa, synthetic construct
GGAGSDLMV

SEQ ID NO: 29424 - protein, 9 aa, synthetic construct
GGAGSDKMY

SEQ ID NO: 29425 - protein, 9 aa, synthetic construct
GGAGSDKVR

SEQ ID NO: 29426 - protein, 9 aa, synthetic construct
GGAGSDKVY

SEQ ID NO: 29427 - protein, 9 aa, synthetic construct
GGAGSDKYI

SEQ ID NO: 29428 - protein, 9 aa, synthetic construct
GGAGSDKYL

SEQ ID NO: 29429 - protein, 9 aa, synthetic construct
GGAGSDLAS

SEQ ID NO: 29430 - protein, 9 aa, synthetic construct
GGAGSDLFA

SEQ ID NO: 29431 - protein, 9 aa, synthetic construct
GGAGSDLFD

SEQ ID NO: 29432 - protein, 9 aa, synthetic construct
GGAGSDLFF

SEQ ID NO: 29433 - protein, 9 aa, synthetic construct
GGAGSDLIA

SEQ ID NO: 29434 - protein, 9 aa, synthetic construct
GGAGSDLIG

SEQ ID NO: 29435 - protein, 9 aa, synthetic construct
GGAGSDLLG

SEQ ID NO: 29436 - protein, 9 aa, synthetic construct
GGAGSDLLH

SEQ ID NO: 29437 - protein, 9 aa, synthetic construct
GGAGSDLLN

SEQ ID NO: 29438 - protein, 9 aa, synthetic construct
GGAGSDLMA

SEQ ID NO: 29439 - protein, 9 aa, synthetic construct
GGAGSDLMF

SEQ ID NO: 29440 - protein, 9 aa, synthetic construct
GGAGSDLMQ

SEQ ID NO: 29441 - protein, 9 aa, synthetic construct
GGAGSDNLL

SEQ ID NO: 29442 - protein, 9 aa, synthetic construct
GGAGSDNLV

SEQ ID NO: 29443 - protein, 9 aa, synthetic construct
GGAGSDNYE

SEQ ID NO: 29444 - protein, 9 aa, synthetic construct
GGAGSDRLA

SEQ ID NO: 29445 - protein, 9 aa, synthetic construct
GGAGSDRLW

SEQ ID NO: 29446 - protein, 9 aa, synthetic construct
GGAGSDRVF

SEQ ID NO: 29447 - protein, 9 aa, synthetic construct
GGAGSDRVN

SEQ ID NO: 29448 - protein, 9 aa, synthetic construct
GGAGSDRVV

SEQ ID NO: 29449 - protein, 9 aa, synthetic construct
GGAGSDRVY

SEQ ID NO: 29450 - protein, 9 aa, synthetic construct
GGAGSDRYY

SEQ ID NO: 29451 - protein, 9 aa, synthetic construct
GGAGSDSAP

SEQ ID NO: 29452 - protein, 9 aa, synthetic construct
GGAGSDSAY

SEQ ID NO: 29453 - protein, 9 aa, synthetic construct
GGAGSDSFD

SEQ ID NO: 29454 - protein, 9 aa, synthetic construct
GGAGSDSFN

SEQ ID NO: 29455 - protein, 9 aa, synthetic construct
GGAGSDSFS

SEQ ID NO: 29456 - protein, 9 aa, synthetic construct
GGAGSDSFT

SEQ ID NO: 29457 - protein, 9 aa, synthetic construct
GGAGSDSIE

SEQ ID NO: 29458 - protein, 9 aa, synthetic construct
GGAGSDSIF

SEQ ID NO: 29459 - protein, 9 aa, synthetic construct
GGAGSDSIH

SEQ ID NO: 29460 - protein, 9 aa, synthetic construct
GGAGSDSII

SEQ ID NO: 29461 - protein, 9 aa, synthetic construct
GGAGSDSIN

SEQ ID NO: 29462 - protein, 9 aa, synthetic construct
GGAGSDRLK

SEQ ID NO: 29463 - protein, 9 aa, synthetic construct
GGAGSDRIQ

SEQ ID NO: 29464 - protein, 9 aa, synthetic construct
GGAGSDNYI

SEQ ID NO: 29465 - protein, 9 aa, synthetic construct
GGAGSDRIM

SEQ ID NO: 29466 - protein, 9 aa, synthetic construct
GGAGSDQAN

SEQ ID NO: 29467 - protein, 9 aa, synthetic construct
GGAGSDQFG

SEQ ID NO: 29468 - protein, 9 aa, synthetic construct
GGAGSDQFI

SEQ ID NO: 29469 - protein, 9 aa, synthetic construct
GGAGSDQFL

SEQ ID NO: 29470 - protein, 9 aa, synthetic construct
GGAGSDQFM

SEQ ID NO: 29471 - protein, 9 aa, synthetic construct
GGAGSDQFN

SEQ ID NO: 29472 - protein, 9 aa, synthetic construct
GGAGSDQID

SEQ ID NO: 29473 - protein, 9 aa, synthetic construct
GGAGSDQIH

SEQ ID NO: 29474 - protein, 9 aa, synthetic construct
GGAGSDQIL

SEQ ID NO: 29475 - protein, 9 aa, synthetic construct
GGAGSDQIR

SEQ ID NO: 29476 - protein, 9 aa, synthetic construct
GGAGSDQIT

SEQ ID NO: 29477 - protein, 9 aa, synthetic construct
GGAGSDQLA

SEQ ID NO: 29478 - protein, 9 aa, synthetic construct
GGAGSDQLW

SEQ ID NO: 29479 - protein, 9 aa, synthetic construct
GGAGSDQMA

SEQ ID NO: 29480 - protein, 9 aa, synthetic construct
GGAGSDQMI

SEQ ID NO: 29481 - protein, 9 aa, synthetic construct
GGAGSDQMN

SEQ ID NO: 29482 - protein, 9 aa, synthetic construct
GGAGSDRIA

SEQ ID NO: 29483 - protein, 9 aa, synthetic construct
GGAGSDKMS

SEQ ID NO: 29484 - protein, 9 aa, synthetic construct
GGAGSDKLN

SEQ ID NO: 29485 - protein, 9 aa, synthetic construct
GGAGSDKLI

SEQ ID NO: 29486 - protein, 9 aa, synthetic construct
GGAGSDEIS

SEQ ID NO: 29487 - protein, 9 aa, synthetic construct
GGAGSDELF

SEQ ID NO: 29488 - protein, 9 aa, synthetic construct
GGAGSDELK

SEQ ID NO: 29489 - protein, 9 aa, synthetic construct
GGAGSDELT

SEQ ID NO: 29490 - protein, 9 aa, synthetic construct
GGAGSDEYH

SEQ ID NO: 29491 - protein, 9 aa, synthetic construct
GGAGSDFAQ

SEQ ID NO: 29492 - protein, 9 aa, synthetic construct
GGAGSDFAS

SEQ ID NO: 29493 - protein, 9 aa, synthetic construct
GGAGSDFAT

SEQ ID NO: 29494 - protein, 9 aa, synthetic construct
GGAGSDFFS

SEQ ID NO: 29495 - protein, 9 aa, synthetic construct
GGAGSDFFV

SEQ ID NO: 29496 - protein, 9 aa, synthetic construct
GGAGSDFID

SEQ ID NO: 29497 - protein, 9 aa, synthetic construct
GGAGSDFIF

SEQ ID NO: 29498 - protein, 9 aa, synthetic construct
GGAGSDFIH

SEQ ID NO: 29499 - protein, 9 aa, synthetic construct
GGAGSDFII

SEQ ID NO: 29500 - protein, 9 aa, synthetic construct
GGAGSDFIM

SEQ ID NO: 29501 - protein, 9 aa, synthetic construct
GGAGSDFIN

SEQ ID NO: 29502 - protein, 9 aa, synthetic construct
GGAGSDFIQ

SEQ ID NO: 29503 - protein, 9 aa, synthetic construct
GGAGSDFIR

SEQ ID NO: 29504 - protein, 9 aa, synthetic construct
GGAGSDEIW

SEQ ID NO: 29505 - protein, 9 aa, synthetic construct
GGAGSDEIQ

SEQ ID NO: 29506 - protein, 9 aa, synthetic construct
GGAGSDFLE

SEQ ID NO: 29507 - protein, 9 aa, synthetic construct
GGAGSDEIN

SEQ ID NO: 29508 - protein, 9 aa, synthetic construct
GGAGSDAYV

SEQ ID NO: 29509 - protein, 9 aa, synthetic construct
GGAGSDCFK

SEQ ID NO: 29510 - protein, 9 aa, synthetic construct
GGAGSDCFV

SEQ ID NO: 29511 - protein, 9 aa, synthetic construct
GGAGSDCID

SEQ ID NO: 29512 - protein, 9 aa, synthetic construct
GGAGSDDID

SEQ ID NO: 29513 - protein, 9 aa, synthetic construct
GGAGSDDIF

SEQ ID NO: 29514 - protein, 9 aa, synthetic construct
GGAGSDDIR

SEQ ID NO: 29515 - protein, 9 aa, synthetic construct
GGAGSDDLE

SEQ ID NO: 29516 - protein, 9 aa, synthetic construct
GGAGSDDLG

SEQ ID NO: 29517 - protein, 9 aa, synthetic construct
GGAGSDDLK

SEQ ID NO: 29518 - protein, 9 aa, synthetic construct
GGAGSDDMK

SEQ ID NO: 29519 - protein, 9 aa, synthetic construct
GGAGSDDVL

SEQ ID NO: 29520 - protein, 9 aa, synthetic construct
GGAGSDDVN

SEQ ID NO: 29521 - protein, 9 aa, synthetic construct
GGAGSDEAL

SEQ ID NO: 29522 - protein, 9 aa, synthetic construct
GGAGSDEFH

SEQ ID NO: 29523 - protein, 9 aa, synthetic construct
GGAGSDEFM

SEQ ID NO: 29524 - protein, 9 aa, synthetic construct
GGAGSDEIH

SEQ ID NO: 29525 - protein, 9 aa, synthetic construct
GGAGSDFIV

SEQ ID NO: 29526 - protein, 9 aa, synthetic construct
GGAGSDFLI

SEQ ID NO: 29527 - protein, 9 aa, synthetic construct
GGAGSDKLA

SEQ ID NO: 29528 - protein, 9 aa, synthetic construct
GGAGSDIFL

SEQ ID NO: 29529 - protein, 9 aa, synthetic construct
GGAGSDIIN

SEQ ID NO: 29530 - protein, 9 aa, synthetic construct
GGAGSDIIR

SEQ ID NO: 29531 - protein, 9 aa, synthetic construct
GGAGSDILG

SEQ ID NO: 29532 - protein, 9 aa, synthetic construct
GGAGSDIMQ

SEQ ID NO: 29533 - protein, 9 aa, synthetic construct
GGAGSDIMT

SEQ ID NO: 29534 - protein, 9 aa, synthetic construct
GGAGSDIMV

SEQ ID NO: 29535 - protein, 9 aa, synthetic construct
GGAGSDIVF

SEQ ID NO: 29536 - protein, 9 aa, synthetic construct
GGAGSDIVL

SEQ ID NO: 29537 - protein, 9 aa, synthetic construct
GGAGSDIVS

SEQ ID NO: 29538 - protein, 9 aa, synthetic construct
GGAGSDIVT

SEQ ID NO: 29539 - protein, 9 aa, synthetic construct
GGAGSDIYN

SEQ ID NO: 29540 - protein, 9 aa, synthetic construct
GGAGSDIYW

SEQ ID NO: 29541 - protein, 9 aa, synthetic construct
GGAGSDKAF

SEQ ID NO: 29542 - protein, 9 aa, synthetic construct
GGAGSDKFK

SEQ ID NO: 29543 - protein, 9 aa, synthetic construct
GGAGSDKFL

SEQ ID NO: 29544 - protein, 9 aa, synthetic construct
GGAGSDKFQ

SEQ ID NO: 29545 - protein, 9 aa, synthetic construct
GGAGSDKFR

SEQ ID NO: 29546 - protein, 9 aa, synthetic construct
GGAGSDIIF

SEQ ID NO: 29547 - protein, 9 aa, synthetic construct
GGAGSDIFE

SEQ ID NO: 29548 - protein, 9 aa, synthetic construct
GGAGSDFLL

SEQ ID NO: 29549 - protein, 9 aa, synthetic construct
GGAGSDIFA

SEQ ID NO: 29550 - protein, 9 aa, synthetic construct
GGAGSDFLY

SEQ ID NO: 29551 - protein, 9 aa, synthetic construct
GGAGSDFMQ

SEQ ID NO: 29552 - protein, 9 aa, synthetic construct
GGAGSDFVF

SEQ ID NO: 29553 - protein, 9 aa, synthetic construct
GGAGSDFVL

SEQ ID NO: 29554 - protein, 9 aa, synthetic construct
GGAGSDGFV

SEQ ID NO: 29555 - protein, 9 aa, synthetic construct
GGAGSDGIF

SEQ ID NO: 29556 - protein, 9 aa, synthetic construct
GGAGSDGIN

SEQ ID NO: 29557 - protein, 9 aa, synthetic construct
GGAGSDGIV

SEQ ID NO: 29558 - protein, 9 aa, synthetic construct
GGAGSDGLG

SEQ ID NO: 29559 - protein, 9 aa, synthetic construct
GGAGSDGLL

SEQ ID NO: 29560 - protein, 9 aa, synthetic construct
GGAGSDGLS

SEQ ID NO: 29561 - protein, 9 aa, synthetic construct
GGAGSDGLT

SEQ ID NO: 29562 - protein, 9 aa, synthetic construct
GGAGSDGYV

SEQ ID NO: 29563 - protein, 9 aa, synthetic construct
GGAGSDHIY

SEQ ID NO: 29564 - protein, 9 aa, synthetic construct
GGAGSDHLR

SEQ ID NO: 29565 - protein, 9 aa, synthetic construct
GGAGSDHVV

SEQ ID NO: 29566 - protein, 9 aa, synthetic construct
GGAGSDIAD

SEQ ID NO: 29567 - protein, 9 aa, synthetic construct
GGAGSDSIQ

SEQ ID NO: 29568 - protein, 9 aa, synthetic construct
GGAGSDSMA

SEQ ID NO: 29569 - protein, 9 aa, synthetic construct
GGAGQDILK

SEQ ID NO: 29570 - protein, 9 aa, synthetic construct
GGAGTDIFV

SEQ ID NO: 29571 - protein, 9 aa, synthetic construct
GGAGTDHIV

SEQ ID NO: 29572 - protein, 9 aa, synthetic construct
GGAGTDHIW

SEQ ID NO: 29573 - protein, 9 aa, synthetic construct
GGAGTDHLT

SEQ ID NO: 29574 - protein, 9 aa, synthetic construct
GGAGTDHMW

SEQ ID NO: 29575 - protein, 9 aa, synthetic construct
GGAGTDHVS

SEQ ID NO: 29576 - protein, 9 aa, synthetic construct
GGAGTDIAI

SEQ ID NO: 29577 - protein, 9 aa, synthetic construct
GGAGTDIFC

SEQ ID NO: 29578 - protein, 9 aa, synthetic construct
GGAGTDIFD

SEQ ID NO: 29579 - protein, 9 aa, synthetic construct
GGAGTDIIQ

SEQ ID NO: 29580 - protein, 9 aa, synthetic construct
GGAGSDSMI

SEQ ID NO: 29581 - protein, 9 aa, synthetic construct
GGAGTDIIY

SEQ ID NO: 29582 - protein, 9 aa, synthetic construct
GGAGTDILF

SEQ ID NO: 29583 - protein, 9 aa, synthetic construct
GGAGTDILG

SEQ ID NO: 29584 - protein, 9 aa, synthetic construct
GGAGTDILH

SEQ ID NO: 29585 - protein, 9 aa, synthetic construct
GGAGTDILY

SEQ ID NO: 29586 - protein, 9 aa, synthetic construct
GGAGTDIMD

SEQ ID NO: 29587 - protein, 9 aa, synthetic construct
GGAGTDIME

SEQ ID NO: 29588 - protein, 9 aa, synthetic construct
GGAGTDIMF

SEQ ID NO: 29589 - protein, 9 aa, synthetic construct
GGAGTDHFW

SEQ ID NO: 29590 - protein, 9 aa, synthetic construct
GGAGTDGLH

SEQ ID NO: 29591 - protein, 9 aa, synthetic construct
GGAGTDGLD

SEQ ID NO: 29592 - protein, 9 aa, synthetic construct
GGAGTDFVS

SEQ ID NO: 29593 - protein, 9 aa, synthetic construct
GGAGTDDMD

SEQ ID NO: 29594 - protein, 9 aa, synthetic construct
GGAGTDDMM

SEQ ID NO: 29595 - protein, 9 aa, synthetic construct
GGAGTDDVD

SEQ ID NO: 29596 - protein, 9 aa, synthetic construct
GGAGTDEFD

SEQ ID NO: 29597 - protein, 9 aa, synthetic construct
GGAGTDEFV

SEQ ID NO: 29598 - protein, 9 aa, synthetic construct
GGAGTDELA

SEQ ID NO: 29599 - protein, 9 aa, synthetic construct
GGAGTDELS

SEQ ID NO: 29600 - protein, 9 aa, synthetic construct
GGAGTDELV

SEQ ID NO: 29601 - protein, 9 aa, synthetic construct
GGAGTDFFR

SEQ ID NO: 29602 - protein, 9 aa, synthetic construct
GGAGTDFIF

SEQ ID NO: 29603 - protein, 9 aa, synthetic construct
GGAGTDFIY

SEQ ID NO: 29604 - protein, 9 aa, synthetic construct
GGAGTDFLF

SEQ ID NO: 29605 - protein, 9 aa, synthetic construct
GGAGTDFLI

SEQ ID NO: 29606 - protein, 9 aa, synthetic construct
GGAGTDFLS

SEQ ID NO: 29607 - protein, 9 aa, synthetic construct
GGAGTDFLV

SEQ ID NO: 29608 - protein, 9 aa, synthetic construct
GGAGTDFLY

SEQ ID NO: 29609 - protein, 9 aa, synthetic construct
GGAGTDFMD

SEQ ID NO: 29610 - protein, 9 aa, synthetic construct
GGAGTDIMN

SEQ ID NO: 29611 - protein, 9 aa, synthetic construct
GGAGTDIVN

SEQ ID NO: 29612 - protein, 9 aa, synthetic construct
GGAGTDIVR

SEQ ID NO: 29613 - protein, 9 aa, synthetic construct
GGAGTDLVV

SEQ ID NO: 29614 - protein, 9 aa, synthetic construct
GGAGTDMVS

SEQ ID NO: 29615 - protein, 9 aa, synthetic construct
GGAGTDNIQ

SEQ ID NO: 29616 - protein, 9 aa, synthetic construct
GGAGTDNLA

SEQ ID NO: 29617 - protein, 9 aa, synthetic construct
GGAGTDNLI

SEQ ID NO: 29618 - protein, 9 aa, synthetic construct
GGAGTDNLL

SEQ ID NO: 29619 - protein, 9 aa, synthetic construct
GGAGTDNMQ

SEQ ID NO: 29620 - protein, 9 aa, synthetic construct
GGAGTDQAF

SEQ ID NO: 29621 - protein, 9 aa, synthetic construct
GGAGTDQIN

SEQ ID NO: 29622 - protein, 9 aa, synthetic construct
GGAGTDQIS

SEQ ID NO: 29623 - protein, 9 aa, synthetic construct
GGAGTDQLA

SEQ ID NO: 29624 - protein, 9 aa, synthetic construct
GGAGTDQLH

SEQ ID NO: 29625 - protein, 9 aa, synthetic construct
GGAGTDQLM

SEQ ID NO: 29626 - protein, 9 aa, synthetic construct
GGAGTDQLN

SEQ ID NO: 29627 - protein, 9 aa, synthetic construct
GGAGTDQLR

SEQ ID NO: 29628 - protein, 9 aa, synthetic construct
GGAGTDQLV

SEQ ID NO: 29629 - protein, 9 aa, synthetic construct
GGAGTDRAM

SEQ ID NO: 29630 - protein, 9 aa, synthetic construct
GGAGTDRAY

SEQ ID NO: 29631 - protein, 9 aa, synthetic construct
GGAGTDMAV

SEQ ID NO: 29632 - protein, 9 aa, synthetic construct
GGAGTDLVT

SEQ ID NO: 29633 - protein, 9 aa, synthetic construct
GGAGTDKIK

SEQ ID NO: 29634 - protein, 9 aa, synthetic construct
GGAGTDLVQ

SEQ ID NO: 29635 - protein, 9 aa, synthetic construct
GGAGTDKLH

SEQ ID NO: 29636 - protein, 9 aa, synthetic construct
GGAGTDKLI

SEQ ID NO: 29637 - protein, 9 aa, synthetic construct
GGAGTDKLL

SEQ ID NO: 29638 - protein, 9 aa, synthetic construct
GGAGTDKMS

SEQ ID NO: 29639 - protein, 9 aa, synthetic construct
GGAGTDKYK

SEQ ID NO: 29640 - protein, 9 aa, synthetic construct
GGAGTDLAD

SEQ ID NO: 29641 - protein, 9 aa, synthetic construct
GGAGTDLAG

SEQ ID NO: 29642 - protein, 9 aa, synthetic construct
GGAGTDLAT

SEQ ID NO: 29643 - protein, 9 aa, synthetic construct
GGAGTDLFF

SEQ ID NO: 29644 - protein, 9 aa, synthetic construct
GGAGTDLFY

SEQ ID NO: 29645 - protein, 9 aa, synthetic construct
GGAGTDLIH

SEQ ID NO: 29646 - protein, 9 aa, synthetic construct
GGAGTDLII

SEQ ID NO: 29647 - protein, 9 aa, synthetic construct
GGAGTDLIY

SEQ ID NO: 29648 - protein, 9 aa, synthetic construct
GGAGTDLLR

SEQ ID NO: 29649 - protein, 9 aa, synthetic construct
GGAGTDLME

SEQ ID NO: 29650 - protein, 9 aa, synthetic construct
GGAGTDLMI

SEQ ID NO: 29651 - protein, 9 aa, synthetic construct
GGAGTDLVF

SEQ ID NO: 29652 - protein, 9 aa, synthetic construct
GGAGTDDLY

SEQ ID NO: 29653 - protein, 9 aa, synthetic construct
GGAGTDDLW

SEQ ID NO: 29654 - protein, 9 aa, synthetic construct
GGAGTDDLL

SEQ ID NO: 29655 - protein, 9 aa, synthetic construct
GGAGSDTVN

SEQ ID NO: 29656 - protein, 9 aa, synthetic construct
GGAGSDTVV

SEQ ID NO: 29657 - protein, 9 aa, synthetic construct
GGAGSDTYH

SEQ ID NO: 29658 - protein, 9 aa, synthetic construct
GGAGSDTYK

SEQ ID NO: 29659 - protein, 9 aa, synthetic construct
GGAGSDTYM

SEQ ID NO: 29660 - protein, 9 aa, synthetic construct
GGAGSDVAL

SEQ ID NO: 29661 - protein, 9 aa, synthetic construct
GGAGSDVAR

SEQ ID NO: 29662 - protein, 9 aa, synthetic construct
GGAGSDVFE

SEQ ID NO: 29663 - protein, 9 aa, synthetic construct
GGAGSDVFI

SEQ ID NO: 29664 - protein, 9 aa, synthetic construct
GGAGSDVFS

SEQ ID NO: 29665 - protein, 9 aa, synthetic construct
GGAGSDVIG

SEQ ID NO: 29666 - protein, 9 aa, synthetic construct
GGAGSDVIL

SEQ ID NO: 29667 - protein, 9 aa, synthetic construct
GGAGSDVIM

SEQ ID NO: 29668 - protein, 9 aa, synthetic construct
GGAGSDVIQ

SEQ ID NO: 29669 - protein, 9 aa, synthetic construct
GGAGSDVIR

SEQ ID NO: 29670 - protein, 9 aa, synthetic construct
GGAGSDVIW

SEQ ID NO: 29671 - protein, 9 aa, synthetic construct
GGAGSDVMF

SEQ ID NO: 29672 - protein, 9 aa, synthetic construct
GGAGSDVMS

SEQ ID NO: 29673 - protein, 9 aa, synthetic construct
GGAGSDTVR

SEQ ID NO: 29674 - protein, 9 aa, synthetic construct
GGAGSDTVI

SEQ ID NO: 29675 - protein, 9 aa, synthetic construct
GGAGSDVVD

SEQ ID NO: 29676 - protein, 9 aa, synthetic construct
GGAGSDTVH

SEQ ID NO: 29677 - protein, 9 aa, synthetic construct
GGAGSDSMQ

SEQ ID NO: 29678 - protein, 9 aa, synthetic construct
GGAGSDSMV

SEQ ID NO: 29679 - protein, 9 aa, synthetic construct
GGAGSDSVA

SEQ ID NO: 29680 - protein, 9 aa, synthetic construct
GGAGSDSVH

SEQ ID NO: 29681 - protein, 9 aa, synthetic construct
GGAGSDSVS

SEQ ID NO: 29682 - protein, 9 aa, synthetic construct
GGAGSDSVT

SEQ ID NO: 29683 - protein, 9 aa, synthetic construct
GGAGSDSVY

SEQ ID NO: 29684 - protein, 9 aa, synthetic construct
GGAGSDSYR

SEQ ID NO: 29685 - protein, 9 aa, synthetic construct
GGAGSDTAA

SEQ ID NO: 29686 - protein, 9 aa, synthetic construct
GGAGSDTAF

SEQ ID NO: 29687 - protein, 9 aa, synthetic construct
GGAGSDTAN

SEQ ID NO: 29688 - protein, 9 aa, synthetic construct
GGAGSDTAT

SEQ ID NO: 29689 - protein, 9 aa, synthetic construct
GGAGSDTFH

SEQ ID NO: 29690 - protein, 9 aa, synthetic construct
GGAGSDTFM

SEQ ID NO: 29691 - protein, 9 aa, synthetic construct
GGAGSDTFY

SEQ ID NO: 29692 - protein, 9 aa, synthetic construct
GGAGSDTIA

SEQ ID NO: 29693 - protein, 9 aa, synthetic construct
GGAGSDTIK

SEQ ID NO: 29694 - protein, 9 aa, synthetic construct
GGAGSDVMV

SEQ ID NO: 29695 - protein, 9 aa, synthetic construct
GGAGSDVVE

SEQ ID NO: 29696 - protein, 9 aa, synthetic construct
GGAGTDDIV

SEQ ID NO: 29697 - protein, 9 aa, synthetic construct
GGAGSDYLI

SEQ ID NO: 29698 - protein, 9 aa, synthetic construct
GGAGSDYLQ

SEQ ID NO: 29699 - protein, 9 aa, synthetic construct
GGAGSDYLW

SEQ ID NO: 29700 - protein, 9 aa, synthetic construct
GGAGSDYVE

SEQ ID NO: 29701 - protein, 9 aa, synthetic construct
GGAGSDYYV

SEQ ID NO: 29702 - protein, 9 aa, synthetic construct
GGAGTDAAD

SEQ ID NO: 29703 - protein, 9 aa, synthetic construct
GGAGTDAAI

SEQ ID NO: 29704 - protein, 9 aa, synthetic construct
GGAGTDAIE

SEQ ID NO: 29705 - protein, 9 aa, synthetic construct
GGAGTDAIR

SEQ ID NO: 29706 - protein, 9 aa, synthetic construct
GGAGTDALA

SEQ ID NO: 29707 - protein, 9 aa, synthetic construct
GGAGTDALD

SEQ ID NO: 29708 - protein, 9 aa, synthetic construct
GGAGTDALE

SEQ ID NO: 29709 - protein, 9 aa, synthetic construct
GGAGTDALF

SEQ ID NO: 29710 - protein, 9 aa, synthetic construct
GGAGTDALS

SEQ ID NO: 29711 - protein, 9 aa, synthetic construct
GGAGTDAMF

SEQ ID NO: 29712 - protein, 9 aa, synthetic construct
GGAGTDAMN

SEQ ID NO: 29713 - protein, 9 aa, synthetic construct
GGAGTDCAV

SEQ ID NO: 29714 - protein, 9 aa, synthetic construct
GGAGTDDFF

SEQ ID NO: 29715 - protein, 9 aa, synthetic construct
GGAGSDYLK

SEQ ID NO: 29716 - protein, 9 aa, synthetic construct
GGAGSDYIV

SEQ ID NO: 29717 - protein, 9 aa, synthetic construct
GGAGSDVVS

SEQ ID NO: 29718 - protein, 9 aa, synthetic construct
GGAGSDYID

SEQ ID NO: 29719 - protein, 9 aa, synthetic construct
GGAGSDVVY

SEQ ID NO: 29720 - protein, 9 aa, synthetic construct
GGAGSDVYA

SEQ ID NO: 29721 - protein, 9 aa, synthetic construct
GGAGSDVYF

SEQ ID NO: 29722 - protein, 9 aa, synthetic construct
GGAGSDVYL

SEQ ID NO: 29723 - protein, 9 aa, synthetic construct
GGAGSDVYT

SEQ ID NO: 29724 - protein, 9 aa, synthetic construct
GGAGSDWAL

SEQ ID NO: 29725 - protein, 9 aa, synthetic construct
GGAGSDWAT

SEQ ID NO: 29726 - protein, 9 aa, synthetic construct
GGAGSDWIS

SEQ ID NO: 29727 - protein, 9 aa, synthetic construct
GGAGSDWLA

SEQ ID NO: 29728 - protein, 9 aa, synthetic construct
GGAGSDWLS

SEQ ID NO: 29729 - protein, 9 aa, synthetic construct
GGAGSDWLV

SEQ ID NO: 29730 - protein, 9 aa, synthetic construct
GGAGSDWMD

SEQ ID NO: 29731 - protein, 9 aa, synthetic construct
GGAGSDWVY

SEQ ID NO: 29732 - protein, 9 aa, synthetic construct
GGAGSDYAD

SEQ ID NO: 29733 - protein, 9 aa, synthetic construct
GGAGSDYAY

SEQ ID NO: 29734 - protein, 9 aa, synthetic construct
GGAGSDYFD

SEQ ID NO: 29735 - protein, 9 aa, synthetic construct
GGAGSDYIA

SEQ ID NO: 29736 - protein, 9 aa, synthetic construct
GGAGSDAYL

SEQ ID NO: 29737 - protein, 9 aa, synthetic construct
GGAGSDAVL

SEQ ID NO: 29738 - protein, 9 aa, synthetic construct
GGAGSDAVG

SEQ ID NO: 29739 - protein, 9 aa, synthetic construct
GGAGRDAIT

SEQ ID NO: 29740 - protein, 9 aa, synthetic construct
GGAGQDYIL

SEQ ID NO: 29741 - protein, 9 aa, synthetic construct
GGAGQDYIS

SEQ ID NO: 29742 - protein, 9 aa, synthetic construct
GGAGRDAFA

SEQ ID NO: 29743 - protein, 9 aa, synthetic construct
GGAGRDAFN

SEQ ID NO: 29744 - protein, 9 aa, synthetic construct
GGAGRDAFY

SEQ ID NO: 29745 - protein, 9 aa, synthetic construct
GGAGRDAIA

SEQ ID NO: 29746 - protein, 9 aa, synthetic construct
GGAGRDAID

SEQ ID NO: 29747 - protein, 9 aa, synthetic construct
GGAGRDAIS

SEQ ID NO: 29748 - protein, 9 aa, synthetic construct
GGAGRDAIW

SEQ ID NO: 29749 - protein, 9 aa, synthetic construct
GGAGSDAMS

SEQ ID NO: 29750 - protein, 9 aa, synthetic construct
GGAGRDALE

SEQ ID NO: 29751 - protein, 9 aa, synthetic construct
GGAGRDALG

SEQ ID NO: 29752 - protein, 9 aa, synthetic construct
GGAGRDALH

SEQ ID NO: 29753 - protein, 9 aa, synthetic construct
GGAGRDALL

SEQ ID NO: 29754 - protein, 9 aa, synthetic construct
GGAGRDALM

SEQ ID NO: 29755 - protein, 9 aa, synthetic construct
GGAGRDALR

SEQ ID NO: 29756 - protein, 9 aa, synthetic construct
GGAGRDAML

SEQ ID NO: 29757 - protein, 9 aa, synthetic construct
GGAGRDAMY

SEQ ID NO: 29758 - protein, 9 aa, synthetic construct
GGAGQDYAD

SEQ ID NO: 29759 - protein, 9 aa, synthetic construct
GGAGQDWVD

SEQ ID NO: 29760 - protein, 9 aa, synthetic construct
GGAGQDWLV

SEQ ID NO: 29761 - protein, 9 aa, synthetic construct
GGAGQDWLD

SEQ ID NO: 29762 - protein, 9 aa, synthetic construct
GGAGQDTMD

SEQ ID NO: 29763 - protein, 9 aa, synthetic construct
GGAGQDTVD

SEQ ID NO: 29764 - protein, 9 aa, synthetic construct
GGAGQDTVI

SEQ ID NO: 29765 - protein, 9 aa, synthetic construct
GGAGQDTVK

SEQ ID NO: 29766 - protein, 9 aa, synthetic construct
GGAGQDTYN

SEQ ID NO: 29767 - protein, 9 aa, synthetic construct
GGAGQDVAE

SEQ ID NO: 29768 - protein, 9 aa, synthetic construct
GGAGQDVFA

SEQ ID NO: 29769 - protein, 9 aa, synthetic construct
GGAGQDVFD

SEQ ID NO: 29770 - protein, 9 aa, synthetic construct
GGAGQDVIE

SEQ ID NO: 29771 - protein, 9 aa, synthetic construct
GGAGQDVIF

SEQ ID NO: 29772 - protein, 9 aa, synthetic construct
GGAGQDVIM

SEQ ID NO: 29773 - protein, 9 aa, synthetic construct
GGAGQDVIY

SEQ ID NO: 29774 - protein, 9 aa, synthetic construct
GGAGQDVLK

SEQ ID NO: 29775 - protein, 9 aa, synthetic construct
GGAGQDVLM

SEQ ID NO: 29776 - protein, 9 aa, synthetic construct
GGAGQDVMR

SEQ ID NO: 29777 - protein, 9 aa, synthetic construct
GGAGQDVMS

SEQ ID NO: 29778 - protein, 9 aa, synthetic construct
GGAGQDVYV

SEQ ID NO: 29779 - protein, 9 aa, synthetic construct
GGAGRDAVD

SEQ ID NO: 29780 - protein, 9 aa, synthetic construct
GGAGRDAVS

SEQ ID NO: 29781 - protein, 9 aa, synthetic construct
GGAGRDDFI

SEQ ID NO: 29782 - protein, 9 aa, synthetic construct
GGAGRDEMR

SEQ ID NO: 29783 - protein, 9 aa, synthetic construct
GGAGRDEVN

SEQ ID NO: 29784 - protein, 9 aa, synthetic construct
GGAGRDFFA

SEQ ID NO: 29785 - protein, 9 aa, synthetic construct
GGAGRDFFV

SEQ ID NO: 29786 - protein, 9 aa, synthetic construct
GGAGRDFIA

SEQ ID NO: 29787 - protein, 9 aa, synthetic construct
GGAGRDFLA

SEQ ID NO: 29788 - protein, 9 aa, synthetic construct
GGAGRDFLI

SEQ ID NO: 29789 - protein, 9 aa, synthetic construct
GGAGRDFLN

SEQ ID NO: 29790 - protein, 9 aa, synthetic construct
GGAGRDFLS

SEQ ID NO: 29791 - protein, 9 aa, synthetic construct
GGAGRDFMS

SEQ ID NO: 29792 - protein, 9 aa, synthetic construct
GGAGRDFVT

SEQ ID NO: 29793 - protein, 9 aa, synthetic construct
GGAGRDFVW

SEQ ID NO: 29794 - protein, 9 aa, synthetic construct
GGAGRDGFE

SEQ ID NO: 29795 - protein, 9 aa, synthetic construct
GGAGRDGIV

SEQ ID NO: 29796 - protein, 9 aa, synthetic construct
GGAGRDGLA

SEQ ID NO: 29797 - protein, 9 aa, synthetic construct
GGAGRDGLE

SEQ ID NO: 29798 - protein, 9 aa, synthetic construct
GGAGRDGLG

SEQ ID NO: 29799 - protein, 9 aa, synthetic construct
GGAGRDGMD

SEQ ID NO: 29800 - protein, 9 aa, synthetic construct
GGAGRDEMT

SEQ ID NO: 29801 - protein, 9 aa, synthetic construct
GGAGRDELF

SEQ ID NO: 29802 - protein, 9 aa, synthetic construct
GGAGRDDID

SEQ ID NO: 29803 - protein, 9 aa, synthetic construct
GGAGRDEIY

SEQ ID NO: 29804 - protein, 9 aa, synthetic construct
GGAGRDDIH

SEQ ID NO: 29805 - protein, 9 aa, synthetic construct
GGAGRDDLE

SEQ ID NO: 29806 - protein, 9 aa, synthetic construct
GGAGRDDLF

SEQ ID NO: 29807 - protein, 9 aa, synthetic construct
GGAGRDDLG

SEQ ID NO: 29808 - protein, 9 aa, synthetic construct
GGAGRDDLS

SEQ ID NO: 29809 - protein, 9 aa, synthetic construct
GGAGRDDLW

SEQ ID NO: 29810 - protein, 9 aa, synthetic construct
GGAGRDDVQ

SEQ ID NO: 29811 - protein, 9 aa, synthetic construct
GGAGRDDVS

SEQ ID NO: 29812 - protein, 9 aa, synthetic construct
GGAGRDDVY

SEQ ID NO: 29813 - protein, 9 aa, synthetic construct
GGAGRDEAA

SEQ ID NO: 29814 - protein, 9 aa, synthetic construct
GGAGRDEAS

SEQ ID NO: 29815 - protein, 9 aa, synthetic construct
GGAGRDEFH

SEQ ID NO: 29816 - protein, 9 aa, synthetic construct
GGAGRDEFL

SEQ ID NO: 29817 - protein, 9 aa, synthetic construct
GGAGRDEFR

SEQ ID NO: 29818 - protein, 9 aa, synthetic construct
GGAGRDEFT

SEQ ID NO: 29819 - protein, 9 aa, synthetic construct
GGAGRDEIH

SEQ ID NO: 29820 - protein, 9 aa, synthetic construct
GGAGRDEIW

SEQ ID NO: 29821 - protein, 9 aa, synthetic construct
GGAGQDTLQ

SEQ ID NO: 29822 - protein, 9 aa, synthetic construct
GGAGQDTLC

SEQ ID NO: 29823 - protein, 9 aa, synthetic construct
GGAGQDTIS

SEQ ID NO: 29824 - protein, 9 aa, synthetic construct
GGAGQDLLY

SEQ ID NO: 29825 - protein, 9 aa, synthetic construct
GGAGQDLMI

SEQ ID NO: 29826 - protein, 9 aa, synthetic construct
GGAGQDLMS

SEQ ID NO: 29827 - protein, 9 aa, synthetic construct
GGAGQDLVE

SEQ ID NO: 29828 - protein, 9 aa, synthetic construct
GGAGQDLVF

SEQ ID NO: 29829 - protein, 9 aa, synthetic construct
GGAGQDLVN

SEQ ID NO: 29830 - protein, 9 aa, synthetic construct
GGAGQDLYL

SEQ ID NO: 29831 - protein, 9 aa, synthetic construct
GGAGQDMAF

SEQ ID NO: 29832 - protein, 9 aa, synthetic construct
GGAGQDMAV

SEQ ID NO: 29833 - protein, 9 aa, synthetic construct
GGAGQDMLD

SEQ ID NO: 29834 - protein, 9 aa, synthetic construct
GGAGQDMLH

SEQ ID NO: 29835 - protein, 9 aa, synthetic construct
GGAGQDMLN

SEQ ID NO: 29836 - protein, 9 aa, synthetic construct
GGAGQDMLS

SEQ ID NO: 29837 - protein, 9 aa, synthetic construct
GGAGQDMLT

SEQ ID NO: 29838 - protein, 9 aa, synthetic construct
GGAGQDMLV

SEQ ID NO: 29839 - protein, 9 aa, synthetic construct
GGAGQDMVF

SEQ ID NO: 29840 - protein, 9 aa, synthetic construct
GGAGQDNAA

SEQ ID NO: 29841 - protein, 9 aa, synthetic construct
GGAGQDNIA

SEQ ID NO: 29842 - protein, 9 aa, synthetic construct
GGAGQDLMF

SEQ ID NO: 29843 - protein, 9 aa, synthetic construct
GGAGQDLLK

SEQ ID NO: 29844 - protein, 9 aa, synthetic construct
GGAGQDNLG

SEQ ID NO: 29845 - protein, 9 aa, synthetic construct
GGAGQDLIW

SEQ ID NO: 29846 - protein, 9 aa, synthetic construct
GGAGQDILL

SEQ ID NO: 29847 - protein, 9 aa, synthetic construct
GGAGQDILV

SEQ ID NO: 29848 - protein, 9 aa, synthetic construct
GGAGQDIMI

SEQ ID NO: 29849 - protein, 9 aa, synthetic construct
GGAGQDKAI

SEQ ID NO: 29850 - protein, 9 aa, synthetic construct
GGAGQDKID

SEQ ID NO: 29851 - protein, 9 aa, synthetic construct
GGAGQDKIN

SEQ ID NO: 29852 - protein, 9 aa, synthetic construct
GGAGQDKIY

SEQ ID NO: 29853 - protein, 9 aa, synthetic construct
GGAGQDKLF

SEQ ID NO: 29854 - protein, 9 aa, synthetic construct
GGAGQDKLS

SEQ ID NO: 29855 - protein, 9 aa, synthetic construct
GGAGQDKLV

SEQ ID NO: 29856 - protein, 9 aa, synthetic construct
GGAGQDKVL

SEQ ID NO: 29857 - protein, 9 aa, synthetic construct
GGAGQDLFI

SEQ ID NO: 29858 - protein, 9 aa, synthetic construct
GGAGQDLFL

SEQ ID NO: 29859 - protein, 9 aa, synthetic construct
GGAGQDLFV

SEQ ID NO: 29860 - protein, 9 aa, synthetic construct
GGAGQDLIF

SEQ ID NO: 29861 - protein, 9 aa, synthetic construct
GGAGQDLIL

SEQ ID NO: 29862 - protein, 9 aa, synthetic construct
GGAGQDLIQ

SEQ ID NO: 29863 - protein, 9 aa, synthetic construct
GGAGQDNLD

SEQ ID NO: 29864 - protein, 9 aa, synthetic construct
GGAGQDNLT

SEQ ID NO: 29865 - protein, 9 aa, synthetic construct
GGAGQDTFS

SEQ ID NO: 29866 - protein, 9 aa, synthetic construct
GGAGQDRME

SEQ ID NO: 29867 - protein, 9 aa, synthetic construct
GGAGQDRVD

SEQ ID NO: 29868 - protein, 9 aa, synthetic construct
GGAGQDRVR

SEQ ID NO: 29869 - protein, 9 aa, synthetic construct
GGAGQDSIR

SEQ ID NO: 29870 - protein, 9 aa, synthetic construct
GGAGQDSLA

SEQ ID NO: 29871 - protein, 9 aa, synthetic construct
GGAGQDSLM

SEQ ID NO: 29872 - protein, 9 aa, synthetic construct
GGAGQDSLN

SEQ ID NO: 29873 - protein, 9 aa, synthetic construct
GGAGQDSLP

SEQ ID NO: 29874 - protein, 9 aa, synthetic construct
GGAGQDSLW

SEQ ID NO: 29875 - protein, 9 aa, synthetic construct
GGAGQDSML

SEQ ID NO: 29876 - protein, 9 aa, synthetic construct
GGAGQDSMN

SEQ ID NO: 29877 - protein, 9 aa, synthetic construct
GGAGQDSMW

SEQ ID NO: 29878 - protein, 9 aa, synthetic construct
GGAGQDSVF

SEQ ID NO: 29879 - protein, 9 aa, synthetic construct
GGAGQDSVH

SEQ ID NO: 29880 - protein, 9 aa, synthetic construct
GGAGQDSVV

SEQ ID NO: 29881 - protein, 9 aa, synthetic construct
GGAGQDTAA

SEQ ID NO: 29882 - protein, 9 aa, synthetic construct
GGAGQDTAD

SEQ ID NO: 29883 - protein, 9 aa, synthetic construct
GGAGQDTFC

SEQ ID NO: 29884 - protein, 9 aa, synthetic construct
GGAGQDRVA

SEQ ID NO: 29885 - protein, 9 aa, synthetic construct
GGAGQDRLV

SEQ ID NO: 29886 - protein, 9 aa, synthetic construct
GGAGQDNVS

SEQ ID NO: 29887 - protein, 9 aa, synthetic construct
GGAGQDRLR

SEQ ID NO: 29888 - protein, 9 aa, synthetic construct
GGAGQDQAR

SEQ ID NO: 29889 - protein, 9 aa, synthetic construct
GGAGQDQID

SEQ ID NO: 29890 - protein, 9 aa, synthetic construct
GGAGQDQIF

SEQ ID NO: 29891 - protein, 9 aa, synthetic construct
GGAGQDQII

SEQ ID NO: 29892 - protein, 9 aa, synthetic construct
GGAGQDQLA

SEQ ID NO: 29893 - protein, 9 aa, synthetic construct
GGAGQDQLH

SEQ ID NO: 29894 - protein, 9 aa, synthetic construct
GGAGQDQLL

SEQ ID NO: 29895 - protein, 9 aa, synthetic construct
GGAGQDQLV

SEQ ID NO: 29896 - protein, 9 aa, synthetic construct
GGAGQDQMS

SEQ ID NO: 29897 - protein, 9 aa, synthetic construct
GGAGQDRAY

SEQ ID NO: 29898 - protein, 9 aa, synthetic construct
GGAGQDRFA

SEQ ID NO: 29899 - protein, 9 aa, synthetic construct
GGAGQDRII

SEQ ID NO: 29900 - protein, 9 aa, synthetic construct
GGAGQDRIL

SEQ ID NO: 29901 - protein, 9 aa, synthetic construct
GGAGQDRIS

SEQ ID NO: 29902 - protein, 9 aa, synthetic construct
GGAGQDRLA

SEQ ID NO: 29903 - protein, 9 aa, synthetic construct
GGAGQDRLN

SEQ ID NO: 29904 - protein, 9 aa, synthetic construct
GGAGQDRLQ

SEQ ID NO: 29905 - protein, 9 aa, synthetic construct
GGAGRDHFM

SEQ ID NO: 29906 - protein, 9 aa, synthetic construct
GGAGRDHFS

SEQ ID NO: 29907 - protein, 9 aa, synthetic construct
GGAGRDHLH

SEQ ID NO: 29908 - protein, 9 aa, synthetic construct
GGAGRDTAD

SEQ ID NO: 29909 - protein, 9 aa, synthetic construct
GGAGRDTAR

SEQ ID NO: 29910 - protein, 9 aa, synthetic construct
GGAGRDTAY

SEQ ID NO: 29911 - protein, 9 aa, synthetic construct
GGAGRDTFD

SEQ ID NO: 29912 - protein, 9 aa, synthetic construct
GGAGRDTFF

SEQ ID NO: 29913 - protein, 9 aa, synthetic construct
GGAGRDTFT

SEQ ID NO: 29914 - protein, 9 aa, synthetic construct
GGAGRDTFY

SEQ ID NO: 29915 - protein, 9 aa, synthetic construct
GGAGRDTIH

SEQ ID NO: 29916 - protein, 9 aa, synthetic construct
GGAGRDTIQ

SEQ ID NO: 29917 - protein, 9 aa, synthetic construct
GGAGRDTMF

SEQ ID NO: 29918 - protein, 9 aa, synthetic construct
GGAGRDTMG

SEQ ID NO: 29919 - protein, 9 aa, synthetic construct
GGAGRDTMN

SEQ ID NO: 29920 - protein, 9 aa, synthetic construct
GGAGRDTVH

SEQ ID NO: 29921 - protein, 9 aa, synthetic construct
GGAGRDTVK

SEQ ID NO: 29922 - protein, 9 aa, synthetic construct
GGAGRDTVQ

SEQ ID NO: 29923 - protein, 9 aa, synthetic construct
GGAGRDTVR

SEQ ID NO: 29924 - protein, 9 aa, synthetic construct
GGAGRDTVT

SEQ ID NO: 29925 - protein, 9 aa, synthetic construct
GGAGRDTYT

SEQ ID NO: 29926 - protein, 9 aa, synthetic construct
GGAGRDTAL

SEQ ID NO: 29927 - protein, 9 aa, synthetic construct
GGAGRDTAA

SEQ ID NO: 29928 - protein, 9 aa, synthetic construct
GGAGRDVAE

SEQ ID NO: 29929 - protein, 9 aa, synthetic construct
GGAGRDSYR

SEQ ID NO: 29930 - protein, 9 aa, synthetic construct
GGAGRDRVE

SEQ ID NO: 29931 - protein, 9 aa, synthetic construct
GGAGRDRVY

SEQ ID NO: 29932 - protein, 9 aa, synthetic construct
GGAGRDRYF

SEQ ID NO: 29933 - protein, 9 aa, synthetic construct
GGAGRDSAN

SEQ ID NO: 29934 - protein, 9 aa, synthetic construct
GGAGRDSFN

SEQ ID NO: 29935 - protein, 9 aa, synthetic construct
GGAGRDSFR

SEQ ID NO: 29936 - protein, 9 aa, synthetic construct
GGAGRDSFY

SEQ ID NO: 29937 - protein, 9 aa, synthetic construct
GGAGRDSIS

SEQ ID NO: 29938 - protein, 9 aa, synthetic construct
GGAGRDSLH

SEQ ID NO: 29939 - protein, 9 aa, synthetic construct
GGAGRDSLK

SEQ ID NO: 29940 - protein, 9 aa, synthetic construct
GGAGRDSLQ

SEQ ID NO: 29941 - protein, 9 aa, synthetic construct
GGAGRDSMA

SEQ ID NO: 29942 - protein, 9 aa, synthetic construct
GGAGRDSMV

SEQ ID NO: 29943 - protein, 9 aa, synthetic construct
GGAGRDSVD

SEQ ID NO: 29944 - protein, 9 aa, synthetic construct
GGAGRDSVL

SEQ ID NO: 29945 - protein, 9 aa, synthetic construct
GGAGRDSVR

SEQ ID NO: 29946 - protein, 9 aa, synthetic construct
GGAGRDSVS

SEQ ID NO: 29947 - protein, 9 aa, synthetic construct
GGAGRDVAD

SEQ ID NO: 29948 - protein, 9 aa, synthetic construct
GGAGRDVAS

SEQ ID NO: 29949 - protein, 9 aa, synthetic construct
GGAGRDRMY

SEQ ID NO: 29950 - protein, 9 aa, synthetic construct
GGAGRDWLV

SEQ ID NO: 29951 - protein, 9 aa, synthetic construct
GGAGRDYFD

SEQ ID NO: 29952 - protein, 9 aa, synthetic construct
GGAGRDYFV

SEQ ID NO: 29953 - protein, 9 aa, synthetic construct
GGAGRDYLF

SEQ ID NO: 29954 - protein, 9 aa, synthetic construct
GGAGRDYLM

SEQ ID NO: 29955 - protein, 9 aa, synthetic construct
GGAGRDYLV

SEQ ID NO: 29956 - protein, 9 aa, synthetic construct
GGAGRDYMW

SEQ ID NO: 29957 - protein, 9 aa, synthetic construct
GGAGRDYVE

SEQ ID NO: 29958 - protein, 9 aa, synthetic construct
GGAGSDAAS

SEQ ID NO: 29959 - protein, 9 aa, synthetic construct
GGAGSDAAY

SEQ ID NO: 29960 - protein, 9 aa, synthetic construct
GGAGSDAFD

SEQ ID NO: 29961 - protein, 9 aa, synthetic construct
GGAGSDAFM

SEQ ID NO: 29962 - protein, 9 aa, synthetic construct
GGAGSDAIA

SEQ ID NO: 29963 - protein, 9 aa, synthetic construct
GGAGSDAIE

SEQ ID NO: 29964 - protein, 9 aa, synthetic construct
GGAGSDALE

SEQ ID NO: 29965 - protein, 9 aa, synthetic construct
GGAGSDALH

SEQ ID NO: 29966 - protein, 9 aa, synthetic construct
GGAGSDALK

SEQ ID NO: 29967 - protein, 9 aa, synthetic construct
GGAGSDAML

SEQ ID NO: 29968 - protein, 9 aa, synthetic construct
GGAGRDYAS

SEQ ID NO: 29969 - protein, 9 aa, synthetic construct
GGAGRDWLQ

SEQ ID NO: 29970 - protein, 9 aa, synthetic construct
GGAGRDVAV

SEQ ID NO: 29971 - protein, 9 aa, synthetic construct
GGAGRDWLG

SEQ ID NO: 29972 - protein, 9 aa, synthetic construct
GGAGRDVFD

SEQ ID NO: 29973 - protein, 9 aa, synthetic construct
GGAGRDVFH

SEQ ID NO: 29974 - protein, 9 aa, synthetic construct
GGAGRDVFM

SEQ ID NO: 29975 - protein, 9 aa, synthetic construct
GGAGRDVFS

SEQ ID NO: 29976 - protein, 9 aa, synthetic construct
GGAGRDVFW

SEQ ID NO: 29977 - protein, 9 aa, synthetic construct
GGAGRDVIE

SEQ ID NO: 29978 - protein, 9 aa, synthetic construct
GGAGRDVIG

SEQ ID NO: 29979 - protein, 9 aa, synthetic construct
GGAGRDVLQ

SEQ ID NO: 29980 - protein, 9 aa, synthetic construct
GGAGRDVME

SEQ ID NO: 29981 - protein, 9 aa, synthetic construct
GGAGRDVVL

SEQ ID NO: 29982 - protein, 9 aa, synthetic construct
GGAGRDVVT

SEQ ID NO: 29983 - protein, 9 aa, synthetic construct
GGAGRDVVV

SEQ ID NO: 29984 - protein, 9 aa, synthetic construct
GGAGRDVYI

SEQ ID NO: 29985 - protein, 9 aa, synthetic construct
GGAGRDVYV

SEQ ID NO: 29986 - protein, 9 aa, synthetic construct
GGAGRDWAR

SEQ ID NO: 29987 - protein, 9 aa, synthetic construct
GGAGRDWAV

SEQ ID NO: 29988 - protein, 9 aa, synthetic construct
GGAGRDWIV

SEQ ID NO: 29989 - protein, 9 aa, synthetic construct
GGAGRDRVD

SEQ ID NO: 29990 - protein, 9 aa, synthetic construct
GGAGRDRMT

SEQ ID NO: 29991 - protein, 9 aa, synthetic construct
GGAGRDHLI

SEQ ID NO: 29992 - protein, 9 aa, synthetic construct
GGAGRDKII

SEQ ID NO: 29993 - protein, 9 aa, synthetic construct
GGAGRDKIS

SEQ ID NO: 29994 - protein, 9 aa, synthetic construct
GGAGRDKLA

SEQ ID NO: 29995 - protein, 9 aa, synthetic construct
GGAGRDKLE

SEQ ID NO: 29996 - protein, 9 aa, synthetic construct
GGAGRDKLW

SEQ ID NO: 29997 - protein, 9 aa, synthetic construct
GGAGRDKML

SEQ ID NO: 29998 - protein, 9 aa, synthetic construct
GGAGRDKVF

SEQ ID NO: 29999 - protein, 9 aa, synthetic construct
GGAGRDLAA

SEQ ID NO: 30000 - protein, 9 aa, synthetic construct
GGAGRDLAQ

SEQ ID NO: 30001 - protein, 9 aa, synthetic construct
GGAGRDLFH

SEQ ID NO: 30002 - protein, 9 aa, synthetic construct
GGAGRDLFI

SEQ ID NO: 30003 - protein, 9 aa, synthetic construct
GGAGRDLFR

SEQ ID NO: 30004 - protein, 9 aa, synthetic construct
GGAGRDLFS

SEQ ID NO: 30005 - protein, 9 aa, synthetic construct
GGAGRDLIA

SEQ ID NO: 30006 - protein, 9 aa, synthetic construct
GGAGRDLIF

SEQ ID NO: 30007 - protein, 9 aa, synthetic construct
GGAGRDLII

SEQ ID NO: 30008 - protein, 9 aa, synthetic construct
GGAGRDLIL

SEQ ID NO: 30009 - protein, 9 aa, synthetic construct
GGAGRDLIT

SEQ ID NO: 30010 - protein, 9 aa, synthetic construct
GGAGRDKIN

SEQ ID NO: 30011 - protein, 9 aa, synthetic construct
GGAGRDKID

SEQ ID NO: 30012 - protein, 9 aa, synthetic construct
GGAGRDLMA

SEQ ID NO: 30013 - protein, 9 aa, synthetic construct
GGAGRDKFV

SEQ ID NO: 30014 - protein, 9 aa, synthetic construct
GGAGRDHLV

SEQ ID NO: 30015 - protein, 9 aa, synthetic construct
GGAGRDHLW

SEQ ID NO: 30016 - protein, 9 aa, synthetic construct
GGAGRDIAI

SEQ ID NO: 30017 - protein, 9 aa, synthetic construct
GGAGRDIFH

SEQ ID NO: 30018 - protein, 9 aa, synthetic construct
GGAGRDIFQ

SEQ ID NO: 30019 - protein, 9 aa, synthetic construct
GGAGRDILE

SEQ ID NO: 30020 - protein, 9 aa, synthetic construct
GGAGRDILH

SEQ ID NO: 30021 - protein, 9 aa, synthetic construct
GGAGRDILY

SEQ ID NO: 30022 - protein, 9 aa, synthetic construct
GGAGRDIMA

SEQ ID NO: 30023 - protein, 9 aa, synthetic construct
GGAGRDIMD

SEQ ID NO: 30024 - protein, 9 aa, synthetic construct
GGAGRDIMR

SEQ ID NO: 30025 - protein, 9 aa, synthetic construct
GGAGRDIMW

SEQ ID NO: 30026 - protein, 9 aa, synthetic construct
GGAGRDIVF

SEQ ID NO: 30027 - protein, 9 aa, synthetic construct
GGAGRDIVN

SEQ ID NO: 30028 - protein, 9 aa, synthetic construct
GGAGRDIYV

SEQ ID NO: 30029 - protein, 9 aa, synthetic construct
GGAGRDKFI

SEQ ID NO: 30030 - protein, 9 aa, synthetic construct
GGAGRDKFL

SEQ ID NO: 30031 - protein, 9 aa, synthetic construct
GGAGRDLLK

SEQ ID NO: 30032 - protein, 9 aa, synthetic construct
GGAGRDLMI

SEQ ID NO: 30033 - protein, 9 aa, synthetic construct
GGAGRDRMN

SEQ ID NO: 30034 - protein, 9 aa, synthetic construct
GGAGRDQFI

SEQ ID NO: 30035 - protein, 9 aa, synthetic construct
GGAGRDQIV

SEQ ID NO: 30036 - protein, 9 aa, synthetic construct
GGAGRDQIW

SEQ ID NO: 30037 - protein, 9 aa, synthetic construct
GGAGRDQLD

SEQ ID NO: 30038 - protein, 9 aa, synthetic construct
GGAGRDQLL

SEQ ID NO: 30039 - protein, 9 aa, synthetic construct
GGAGRDQLN

SEQ ID NO: 30040 - protein, 9 aa, synthetic construct
GGAGRDQLY

SEQ ID NO: 30041 - protein, 9 aa, synthetic construct
GGAGRDQMF

SEQ ID NO: 30042 - protein, 9 aa, synthetic construct
GGAGRDRAH

SEQ ID NO: 30043 - protein, 9 aa, synthetic construct
GGAGRDRAL

SEQ ID NO: 30044 - protein, 9 aa, synthetic construct
GGAGRDRFE

SEQ ID NO: 30045 - protein, 9 aa, synthetic construct
GGAGRDRFI

SEQ ID NO: 30046 - protein, 9 aa, synthetic construct
GGAGRDRFY

SEQ ID NO: 30047 - protein, 9 aa, synthetic construct
GGAGRDRIE

SEQ ID NO: 30048 - protein, 9 aa, synthetic construct
GGAGRDRIF

SEQ ID NO: 30049 - protein, 9 aa, synthetic construct
GGAGRDRIG

SEQ ID NO: 30050 - protein, 9 aa, synthetic construct
GGAGRDRIT

SEQ ID NO: 30051 - protein, 9 aa, synthetic construct
GGAGRDRLM

SEQ ID NO: 30052 - protein, 9 aa, synthetic construct
GGAGRDQFT

SEQ ID NO: 30053 - protein, 9 aa, synthetic construct
GGAGRDQFD

SEQ ID NO: 30054 - protein, 9 aa, synthetic construct
GGAGRDLMQ

SEQ ID NO: 30055 - protein, 9 aa, synthetic construct
GGAGRDNMT

SEQ ID NO: 30056 - protein, 9 aa, synthetic construct
GGAGRDLMT

SEQ ID NO: 30057 - protein, 9 aa, synthetic construct
GGAGRDLVH

SEQ ID NO: 30058 - protein, 9 aa, synthetic construct
GGAGRDLVL

SEQ ID NO: 30059 - protein, 9 aa, synthetic construct
GGAGRDLVS

SEQ ID NO: 30060 - protein, 9 aa, synthetic construct
GGAGRDMFV

SEQ ID NO: 30061 - protein, 9 aa, synthetic construct
GGAGRDMII

SEQ ID NO: 30062 - protein, 9 aa, synthetic construct
GGAGRDMLI

SEQ ID NO: 30063 - protein, 9 aa, synthetic construct
GGAGRDMLK

SEQ ID NO: 30064 - protein, 9 aa, synthetic construct
GGAGRDMVL

SEQ ID NO: 30065 - protein, 9 aa, synthetic construct
GGAGRDMVS

SEQ ID NO: 30066 - protein, 9 aa, synthetic construct
GGAGRDNFV

SEQ ID NO: 30067 - protein, 9 aa, synthetic construct
GGAGRDNID

SEQ ID NO: 30068 - protein, 9 aa, synthetic construct
GGAGRDNIG

SEQ ID NO: 30069 - protein, 9 aa, synthetic construct
GGAGRDNIQ

SEQ ID NO: 30070 - protein, 9 aa, synthetic construct
GGAGRDNLH

SEQ ID NO: 30071 - protein, 9 aa, synthetic construct
GGAGRDNLQ

SEQ ID NO: 30072 - protein, 9 aa, synthetic construct
GGAGRDNLR

SEQ ID NO: 30073 - protein, 9 aa, synthetic construct
GGAGKDIMV

SEQ ID NO: 30074 - protein, 9 aa, synthetic construct
GGAGKDIMR

SEQ ID NO: 30075 - protein, 9 aa, synthetic construct
GGAGKDIMI

SEQ ID NO: 30076 - protein, 9 aa, synthetic construct
GGAGDDQFV

SEQ ID NO: 30077 - protein, 9 aa, synthetic construct
GGAGDDNMG

SEQ ID NO: 30078 - protein, 9 aa, synthetic construct
GGAGDDNMI

SEQ ID NO: 30079 - protein, 9 aa, synthetic construct
GGAGDDNVS

SEQ ID NO: 30080 - protein, 9 aa, synthetic construct
GGAGDDNVT

SEQ ID NO: 30081 - protein, 9 aa, synthetic construct
GGAGDDNYF

SEQ ID NO: 30082 - protein, 9 aa, synthetic construct
GGAGDDQAH

SEQ ID NO: 30083 - protein, 9 aa, synthetic construct
GGAGDDQFF

SEQ ID NO: 30084 - protein, 9 aa, synthetic construct
GGAGDDQFI

SEQ ID NO: 30085 - protein, 9 aa, synthetic construct
GGAGDDQFY

SEQ ID NO: 30086 - protein, 9 aa, synthetic construct
GGAGDDSVF

SEQ ID NO: 30087 - protein, 9 aa, synthetic construct
GGAGDDQIE

SEQ ID NO: 30088 - protein, 9 aa, synthetic construct
GGAGDDQIM

SEQ ID NO: 30089 - protein, 9 aa, synthetic construct
GGAGDDQIW

SEQ ID NO: 30090 - protein, 9 aa, synthetic construct
GGAGDDQMA

SEQ ID NO: 30091 - protein, 9 aa, synthetic construct
GGAGDDQMD

SEQ ID NO: 30092 - protein, 9 aa, synthetic construct
GGAGDDQME

SEQ ID NO: 30093 - protein, 9 aa, synthetic construct
GGAGDDQMF

SEQ ID NO: 30094 - protein, 9 aa, synthetic construct
GGAGDDQMG

SEQ ID NO: 30095 - protein, 9 aa, synthetic construct
GGAGDDNLM

SEQ ID NO: 30096 - protein, 9 aa, synthetic construct
GGAGDDNLI

SEQ ID NO: 30097 - protein, 9 aa, synthetic construct
GGAGDDNLE

SEQ ID NO: 30098 - protein, 9 aa, synthetic construct
GGAGDDNIY

SEQ ID NO: 30099 - protein, 9 aa, synthetic construct
GGAGDDMLK

SEQ ID NO: 30100 - protein, 9 aa, synthetic construct
GGAGDDMLW

SEQ ID NO: 30101 - protein, 9 aa, synthetic construct
GGAGDDMMA

SEQ ID NO: 30102 - protein, 9 aa, synthetic construct
GGAGDDMMR

SEQ ID NO: 30103 - protein, 9 aa, synthetic construct
GGAGDDMMS

SEQ ID NO: 30104 - protein, 9 aa, synthetic construct
GGAGDDMMT

SEQ ID NO: 30105 - protein, 9 aa, synthetic construct
GGAGDDMVD

SEQ ID NO: 30106 - protein, 9 aa, synthetic construct
GGAGDDMVN

SEQ ID NO: 30107 - protein, 9 aa, synthetic construct
GGAGDDMVT

SEQ ID NO: 30108 - protein, 9 aa, synthetic construct
GGAGDDMYI

SEQ ID NO: 30109 - protein, 9 aa, synthetic construct
GGAGDDNAD

SEQ ID NO: 30110 - protein, 9 aa, synthetic construct
GGAGDDNFI

SEQ ID NO: 30111 - protein, 9 aa, synthetic construct
GGAGDDNIE

SEQ ID NO: 30112 - protein, 9 aa, synthetic construct
GGAGDDNIK

SEQ ID NO: 30113 - protein, 9 aa, synthetic construct
GGAGDDNIM

SEQ ID NO: 30114 - protein, 9 aa, synthetic construct
GGAGDDNIN

SEQ ID NO: 30115 - protein, 9 aa, synthetic construct
GGAGDDNIT

SEQ ID NO: 30116 - protein, 9 aa, synthetic construct
GGAGDDQMI

SEQ ID NO: 30117 - protein, 9 aa, synthetic construct
GGAGDDQMN

SEQ ID NO: 30118 - protein, 9 aa, synthetic construct
GGAGDDQMS

SEQ ID NO: 30119 - protein, 9 aa, synthetic construct
GGAGDDSAI

SEQ ID NO: 30120 - protein, 9 aa, synthetic construct
GGAGDDSAV

SEQ ID NO: 30121 - protein, 9 aa, synthetic construct
GGAGDDSFF

SEQ ID NO: 30122 - protein, 9 aa, synthetic construct
GGAGDDSFK

SEQ ID NO: 30123 - protein, 9 aa, synthetic construct
GGAGDDSFM

SEQ ID NO: 30124 - protein, 9 aa, synthetic construct
GGAGDDSFN

SEQ ID NO: 30125 - protein, 9 aa, synthetic construct
GGAGDDSFV

SEQ ID NO: 30126 - protein, 9 aa, synthetic construct
GGAGDDSFW

SEQ ID NO: 30127 - protein, 9 aa, synthetic construct
GGAGDDSFY

SEQ ID NO: 30128 - protein, 9 aa, synthetic construct
GGAGDDSIK

SEQ ID NO: 30129 - protein, 9 aa, synthetic construct
GGAGDDSIM

SEQ ID NO: 30130 - protein, 9 aa, synthetic construct
GGAGDDSIW

SEQ ID NO: 30131 - protein, 9 aa, synthetic construct
GGAGDDSLC

SEQ ID NO: 30132 - protein, 9 aa, synthetic construct
GGAGDDSML

SEQ ID NO: 30133 - protein, 9 aa, synthetic construct
GGAGDDSMQ

SEQ ID NO: 30134 - protein, 9 aa, synthetic construct
GGAGDDSMR

SEQ ID NO: 30135 - protein, 9 aa, synthetic construct
GGAGDDSMT

SEQ ID NO: 30136 - protein, 9 aa, synthetic construct
GGAGDDSMY

SEQ ID NO: 30137 - protein, 9 aa, synthetic construct
GGAGDDSAS

SEQ ID NO: 30138 - protein, 9 aa, synthetic construct
GGAGDDSAD

SEQ ID NO: 30139 - protein, 9 aa, synthetic construct
GGAGDDQVH

SEQ ID NO: 30140 - protein, 9 aa, synthetic construct
GGAGDDRVW

SEQ ID NO: 30141 - protein, 9 aa, synthetic construct
GGAGDDQVK

SEQ ID NO: 30142 - protein, 9 aa, synthetic construct
GGAGDDQVR

SEQ ID NO: 30143 - protein, 9 aa, synthetic construct
GGAGDDQVS

SEQ ID NO: 30144 - protein, 9 aa, synthetic construct
GGAGDDQYQ

SEQ ID NO: 30145 - protein, 9 aa, synthetic construct
GGAGDDQYR

SEQ ID NO: 30146 - protein, 9 aa, synthetic construct
GGAGDDRAF

SEQ ID NO: 30147 - protein, 9 aa, synthetic construct
GGAGDDRAI

SEQ ID NO: 30148 - protein, 9 aa, synthetic construct
GGAGDDRAN

SEQ ID NO: 30149 - protein, 9 aa, synthetic construct
GGAGDDRAR

SEQ ID NO: 30150 - protein, 9 aa, synthetic construct
GGAGDDRAT

SEQ ID NO: 30151 - protein, 9 aa, synthetic construct
GGAGDDRIG

SEQ ID NO: 30152 - protein, 9 aa, synthetic construct
GGAGDDRIH

SEQ ID NO: 30153 - protein, 9 aa, synthetic construct
GGAGDDRML

SEQ ID NO: 30154 - protein, 9 aa, synthetic construct
GGAGDDRMV

SEQ ID NO: 30155 - protein, 9 aa, synthetic construct
GGAGDDRVM

SEQ ID NO: 30156 - protein, 9 aa, synthetic construct
GGAGDDRVN

SEQ ID NO: 30157 - protein, 9 aa, synthetic construct
GGAGDDRVV

SEQ ID NO: 30158 - protein, 9 aa, synthetic construct
GGAGDDMLH

SEQ ID NO: 30159 - protein, 9 aa, synthetic construct
GGAGDDMLG

SEQ ID NO: 30160 - protein, 9 aa, synthetic construct
GGAGDDMIN

SEQ ID NO: 30161 - protein, 9 aa, synthetic construct
GGAGDDHYI

SEQ ID NO: 30162 - protein, 9 aa, synthetic construct
GGAGDDIAL

SEQ ID NO: 30163 - protein, 9 aa, synthetic construct
GGAGDDIAR

SEQ ID NO: 30164 - protein, 9 aa, synthetic construct
GGAGDDIAS

SEQ ID NO: 30165 - protein, 9 aa, synthetic construct
GGAGDDIAV

SEQ ID NO: 30166 - protein, 9 aa, synthetic construct
GGAGDDIAW

SEQ ID NO: 30167 - protein, 9 aa, synthetic construct
GGAGDDIFA

SEQ ID NO: 30168 - protein, 9 aa, synthetic construct
GGAGDDIFH

SEQ ID NO: 30169 - protein, 9 aa, synthetic construct
GGAGDDIFI

SEQ ID NO: 30170 - protein, 9 aa, synthetic construct
GGAGDDIFQ

SEQ ID NO: 30171 - protein, 9 aa, synthetic construct
GGAGDDIFS

SEQ ID NO: 30172 - protein, 9 aa, synthetic construct
GGAGDDIIC

SEQ ID NO: 30173 - protein, 9 aa, synthetic construct
GGAGDDIIW

SEQ ID NO: 30174 - protein, 9 aa, synthetic construct
GGAGDDIIX

SEQ ID NO: 30175 - protein, 9 aa, synthetic construct
GGAGDDILC

SEQ ID NO: 30176 - protein, 9 aa, synthetic construct
GGAGDDIMH

SEQ ID NO: 30177 - protein, 9 aa, synthetic construct
GGAGDDIML

SEQ ID NO: 30178 - protein, 9 aa, synthetic construct
GGAGDDIMN

SEQ ID NO: 30179 - protein, 9 aa, synthetic construct
GGAGDDHYV

SEQ ID NO: 30180 - protein, 9 aa, synthetic construct
GGAGDDHVN

SEQ ID NO: 30181 - protein, 9 aa, synthetic construct
GGAGDDIVV

SEQ ID NO: 30182 - protein, 9 aa, synthetic construct
GGAGDDHVI

SEQ ID NO: 30183 - protein, 9 aa, synthetic construct
GGAGDDGLH

SEQ ID NO: 30184 - protein, 9 aa, synthetic construct
GGAGDDGLM

SEQ ID NO: 30185 - protein, 9 aa, synthetic construct
GGAGDDGLW

SEQ ID NO: 30186 - protein, 9 aa, synthetic construct
GGAGDDGVF

SEQ ID NO: 30187 - protein, 9 aa, synthetic construct
GGAGDDGYE

SEQ ID NO: 30188 - protein, 9 aa, synthetic construct
GGAGDDHAD

SEQ ID NO: 30189 - protein, 9 aa, synthetic construct
GGAGDDHAN

SEQ ID NO: 30190 - protein, 9 aa, synthetic construct
GGAGDDHFF

SEQ ID NO: 30191 - protein, 9 aa, synthetic construct
GGAGDDHFI

SEQ ID NO: 30192 - protein, 9 aa, synthetic construct
GGAGDDHIA

SEQ ID NO: 30193 - protein, 9 aa, synthetic construct
GGAGDDHIG

SEQ ID NO: 30194 - protein, 9 aa, synthetic construct
GGAGDDHIT

SEQ ID NO: 30195 - protein, 9 aa, synthetic construct
GGAGDDHIY

SEQ ID NO: 30196 - protein, 9 aa, synthetic construct
GGAGDDHMA

SEQ ID NO: 30197 - protein, 9 aa, synthetic construct
GGAGDDHME

SEQ ID NO: 30198 - protein, 9 aa, synthetic construct
GGAGDDHMQ

SEQ ID NO: 30199 - protein, 9 aa, synthetic construct
GGAGDDHMT

SEQ ID NO: 30200 - protein, 9 aa, synthetic construct
GGAGDDIMV

SEQ ID NO: 30201 - protein, 9 aa, synthetic construct
GGAGDDIYW

SEQ ID NO: 30202 - protein, 9 aa, synthetic construct
GGAGDDMIM

SEQ ID NO: 30203 - protein, 9 aa, synthetic construct
GGAGDDLAQ

SEQ ID NO: 30204 - protein, 9 aa, synthetic construct
GGAGDDLFA

SEQ ID NO: 30205 - protein, 9 aa, synthetic construct
GGAGDDLFD

SEQ ID NO: 30206 - protein, 9 aa, synthetic construct
GGAGDDLFH

SEQ ID NO: 30207 - protein, 9 aa, synthetic construct
GGAGDDLFQ

SEQ ID NO: 30208 - protein, 9 aa, synthetic construct
GGAGDDLFS

SEQ ID NO: 30209 - protein, 9 aa, synthetic construct
GGAGDDLFT

SEQ ID NO: 30210 - protein, 9 aa, synthetic construct
GGAGDDLMK

SEQ ID NO: 30211 - protein, 9 aa, synthetic construct
GGAGDDLMS

SEQ ID NO: 30212 - protein, 9 aa, synthetic construct
GGAGDDLMV

SEQ ID NO: 30213 - protein, 9 aa, synthetic construct
GGAGDDLVH

SEQ ID NO: 30214 - protein, 9 aa, synthetic construct
GGAGDDLVW

SEQ ID NO: 30215 - protein, 9 aa, synthetic construct
GGAGDDLYD

SEQ ID NO: 30216 - protein, 9 aa, synthetic construct
GGAGDDLYE

SEQ ID NO: 30217 - protein, 9 aa, synthetic construct
GGAGDDMFA

SEQ ID NO: 30218 - protein, 9 aa, synthetic construct
GGAGDDMFY

SEQ ID NO: 30219 - protein, 9 aa, synthetic construct
GGAGDDMII

SEQ ID NO: 30220 - protein, 9 aa, synthetic construct
GGAGDDMIK

SEQ ID NO: 30221 - protein, 9 aa, synthetic construct
GGAGDDLAY

SEQ ID NO: 30222 - protein, 9 aa, synthetic construct
GGAGDDLAN

SEQ ID NO: 30223 - protein, 9 aa, synthetic construct
GGAGDDKFI

SEQ ID NO: 30224 - protein, 9 aa, synthetic construct
GGAGDDLAG

SEQ ID NO: 30225 - protein, 9 aa, synthetic construct
GGAGDDKFY

SEQ ID NO: 30226 - protein, 9 aa, synthetic construct
GGAGDDKIE

SEQ ID NO: 30227 - protein, 9 aa, synthetic construct
GGAGDDKIG

SEQ ID NO: 30228 - protein, 9 aa, synthetic construct
GGAGDDKIH

SEQ ID NO: 30229 - protein, 9 aa, synthetic construct
GGAGDDKIL

SEQ ID NO: 30230 - protein, 9 aa, synthetic construct
GGAGDDKIS

SEQ ID NO: 30231 - protein, 9 aa, synthetic construct
GGAGDDKLK

SEQ ID NO: 30232 - protein, 9 aa, synthetic construct
GGAGDDKLQ

SEQ ID NO: 30233 - protein, 9 aa, synthetic construct
GGAGDDKMD

SEQ ID NO: 30234 - protein, 9 aa, synthetic construct
GGAGDDKMK

SEQ ID NO: 30235 - protein, 9 aa, synthetic construct
GGAGDDKML

SEQ ID NO: 30236 - protein, 9 aa, synthetic construct
GGAGDDKVD

SEQ ID NO: 30237 - protein, 9 aa, synthetic construct
GGAGDDKVI

SEQ ID NO: 30238 - protein, 9 aa, synthetic construct
GGAGDDKVS

SEQ ID NO: 30239 - protein, 9 aa, synthetic construct
GGAGDDKVV

SEQ ID NO: 30240 - protein, 9 aa, synthetic construct
GGAGDDKVY

SEQ ID NO: 30241 - protein, 9 aa, synthetic construct
GGAGDDLAF

SEQ ID NO: 30242 - protein, 9 aa, synthetic construct
GGAGDDSVA

SEQ ID NO: 30243 - protein, 9 aa, synthetic construct
GGAGDDSVG

SEQ ID NO: 30244 - protein, 9 aa, synthetic construct
GGAGEDTMT

SEQ ID NO: 30245 - protein, 9 aa, synthetic construct
GGAGEDMLV

SEQ ID NO: 30246 - protein, 9 aa, synthetic construct
GGAGEDLIS

SEQ ID NO: 30247 - protein, 9 aa, synthetic construct
GGAGEDLLF

SEQ ID NO: 30248 - protein, 9 aa, synthetic construct
GGAGEDLVW

SEQ ID NO: 30249 - protein, 9 aa, synthetic construct
GGAGEDMAD

SEQ ID NO: 30250 - protein, 9 aa, synthetic construct
GGAGEDMID

SEQ ID NO: 30251 - protein, 9 aa, synthetic construct
GGAGEDMIN

SEQ ID NO: 30252 - protein, 9 aa, synthetic construct
GGAGEDMLI

SEQ ID NO: 30253 - protein, 9 aa, synthetic construct
GGAGEDMLS

SEQ ID NO: 30254 - protein, 9 aa, synthetic construct
GGAGEDMLY

SEQ ID NO: 30255 - protein, 9 aa, synthetic construct
GGAGDDSVN

SEQ ID NO: 30256 - protein, 9 aa, synthetic construct
GGAGEDNIQ

SEQ ID NO: 30257 - protein, 9 aa, synthetic construct
GGAGEDNIT

SEQ ID NO: 30258 - protein, 9 aa, synthetic construct
GGAGEDNLD

SEQ ID NO: 30259 - protein, 9 aa, synthetic construct
GGAGEDNLI

SEQ ID NO: 30260 - protein, 9 aa, synthetic construct
GGAGEDQIA

SEQ ID NO: 30261 - protein, 9 aa, synthetic construct
GGAGEDQIF

SEQ ID NO: 30262 - protein, 9 aa, synthetic construct
GGAGEDQIR

SEQ ID NO: 30263 - protein, 9 aa, synthetic construct
GGAGEDQIT

SEQ ID NO: 30264 - protein, 9 aa, synthetic construct
GGAGEDLIN

SEQ ID NO: 30265 - protein, 9 aa, synthetic construct
GGAGEDLIE

SEQ ID NO: 30266 - protein, 9 aa, synthetic construct
GGAGEDLFI

SEQ ID NO: 30267 - protein, 9 aa, synthetic construct
GGAGEDKLW

SEQ ID NO: 30268 - protein, 9 aa, synthetic construct
GGAGEDGIG

SEQ ID NO: 30269 - protein, 9 aa, synthetic construct
GGAGEDGIL

SEQ ID NO: 30270 - protein, 9 aa, synthetic construct
GGAGEDGLA

SEQ ID NO: 30271 - protein, 9 aa, synthetic construct
GGAGEDGMT

SEQ ID NO: 30272 - protein, 9 aa, synthetic construct
GGAGEDHID

SEQ ID NO: 30273 - protein, 9 aa, synthetic construct
GGAGEDHLD

SEQ ID NO: 30274 - protein, 9 aa, synthetic construct
GGAGEDHLS

SEQ ID NO: 30275 - protein, 9 aa, synthetic construct
GGAGEDIFE

SEQ ID NO: 30276 - protein, 9 aa, synthetic construct
GGAGEDIFI

SEQ ID NO: 30277 - protein, 9 aa, synthetic construct
GGAGEDILE

SEQ ID NO: 30278 - protein, 9 aa, synthetic construct
GGAGEDILH

SEQ ID NO: 30279 - protein, 9 aa, synthetic construct
GGAGEDILK

SEQ ID NO: 30280 - protein, 9 aa, synthetic construct
GGAGEDIVA

SEQ ID NO: 30281 - protein, 9 aa, synthetic construct
GGAGEDIVE

SEQ ID NO: 30282 - protein, 9 aa, synthetic construct
GGAGEDKAE

SEQ ID NO: 30283 - protein, 9 aa, synthetic construct
GGAGEDKID

SEQ ID NO: 30284 - protein, 9 aa, synthetic construct
GGAGEDKLD

SEQ ID NO: 30285 - protein, 9 aa, synthetic construct
GGAGEDQLI

SEQ ID NO: 30286 - protein, 9 aa, synthetic construct
GGAGEDQLV

SEQ ID NO: 30287 - protein, 9 aa, synthetic construct
GGAGEDQMH

SEQ ID NO: 30288 - protein, 9 aa, synthetic construct
GGAGEDSIV

SEQ ID NO: 30289 - protein, 9 aa, synthetic construct
GGAGEDSLT

SEQ ID NO: 30290 - protein, 9 aa, synthetic construct
GGAGEDSLV

SEQ ID NO: 30291 - protein, 9 aa, synthetic construct
GGAGEDSLY

SEQ ID NO: 30292 - protein, 9 aa, synthetic construct
GGAGEDSVT

SEQ ID NO: 30293 - protein, 9 aa, synthetic construct
GGAGEDTAI

SEQ ID NO: 30294 - protein, 9 aa, synthetic construct
GGAGEDTAN

SEQ ID NO: 30295 - protein, 9 aa, synthetic construct
GGAGEDTFG

SEQ ID NO: 30296 - protein, 9 aa, synthetic construct
GGAGEDTIA

SEQ ID NO: 30297 - protein, 9 aa, synthetic construct
GGAGEDTII

SEQ ID NO: 30298 - protein, 9 aa, synthetic construct
GGAGEDTIT

SEQ ID NO: 30299 - protein, 9 aa, synthetic construct
GGAGEDTIV

SEQ ID NO: 30300 - protein, 9 aa, synthetic construct
GGAGEDTIY

SEQ ID NO: 30301 - protein, 9 aa, synthetic construct
GGAGEDTLM

SEQ ID NO: 30302 - protein, 9 aa, synthetic construct
GGAGEDTLR

SEQ ID NO: 30303 - protein, 9 aa, synthetic construct
GGAGEDTMD

SEQ ID NO: 30304 - protein, 9 aa, synthetic construct
GGAGEDTME

SEQ ID NO: 30305 - protein, 9 aa, synthetic construct
GGAGEDTML

SEQ ID NO: 30306 - protein, 9 aa, synthetic construct
GGAGEDSLE

SEQ ID NO: 30307 - protein, 9 aa, synthetic construct
GGAGEDSIT

SEQ ID NO: 30308 - protein, 9 aa, synthetic construct
GGAGEDQVS

SEQ ID NO: 30309 - protein, 9 aa, synthetic construct
GGAGEDSIR

SEQ ID NO: 30310 - protein, 9 aa, synthetic construct
GGAGEDRFD

SEQ ID NO: 30311 - protein, 9 aa, synthetic construct
GGAGEDRFV

SEQ ID NO: 30312 - protein, 9 aa, synthetic construct
GGAGEDRIA

SEQ ID NO: 30313 - protein, 9 aa, synthetic construct
GGAGEDRIL

SEQ ID NO: 30314 - protein, 9 aa, synthetic construct
GGAGEDRIY

SEQ ID NO: 30315 - protein, 9 aa, synthetic construct
GGAGEDRLR

SEQ ID NO: 30316 - protein, 9 aa, synthetic construct
GGAGEDRME

SEQ ID NO: 30317 - protein, 9 aa, synthetic construct
GGAGEDRMI

SEQ ID NO: 30318 - protein, 9 aa, synthetic construct
GGAGEDRMT

SEQ ID NO: 30319 - protein, 9 aa, synthetic construct
GGAGEDRVH

SEQ ID NO: 30320 - protein, 9 aa, synthetic construct
GGAGEDRVS

SEQ ID NO: 30321 - protein, 9 aa, synthetic construct
GGAGEDRYV

SEQ ID NO: 30322 - protein, 9 aa, synthetic construct
GGAGEDSFL

SEQ ID NO: 30323 - protein, 9 aa, synthetic construct
GGAGEDSFR

SEQ ID NO: 30324 - protein, 9 aa, synthetic construct
GGAGEDSFV

SEQ ID NO: 30325 - protein, 9 aa, synthetic construct
GGAGEDSFY

SEQ ID NO: 30326 - protein, 9 aa, synthetic construct
GGAGEDSID

SEQ ID NO: 30327 - protein, 9 aa, synthetic construct
GGAGEDFVS

SEQ ID NO: 30328 - protein, 9 aa, synthetic construct
GGAGEDFVK

SEQ ID NO: 30329 - protein, 9 aa, synthetic construct
GGAGEDFLQ

SEQ ID NO: 30330 - protein, 9 aa, synthetic construct
GGAGDDVFM

SEQ ID NO: 30331 - protein, 9 aa, synthetic construct
GGAGDDVIM

SEQ ID NO: 30332 - protein, 9 aa, synthetic construct
GGAGDDVVH

SEQ ID NO: 30333 - protein, 9 aa, synthetic construct
GGAGDDVYM

SEQ ID NO: 30334 - protein, 9 aa, synthetic construct
GGAGDDVYS

SEQ ID NO: 30335 - protein, 9 aa, synthetic construct
GGAGDDVYT

SEQ ID NO: 30336 - protein, 9 aa, synthetic construct
GGAGDDWAL

SEQ ID NO: 30337 - protein, 9 aa, synthetic construct
GGAGDDWFE

SEQ ID NO: 30338 - protein, 9 aa, synthetic construct
GGAGDDWFI

SEQ ID NO: 30339 - protein, 9 aa, synthetic construct
GGAGDDWII

SEQ ID NO: 30340 - protein, 9 aa, synthetic construct
GGAGDDWIQ

SEQ ID NO: 30341 - protein, 9 aa, synthetic construct
GGAGDDWIR

SEQ ID NO: 30342 - protein, 9 aa, synthetic construct
GGAGDDWIT

SEQ ID NO: 30343 - protein, 9 aa, synthetic construct
GGAGDDWIY

SEQ ID NO: 30344 - protein, 9 aa, synthetic construct
GGAGDDWLG

SEQ ID NO: 30345 - protein, 9 aa, synthetic construct
GGAGDDWMA

SEQ ID NO: 30346 - protein, 9 aa, synthetic construct
GGAGDDWMD

SEQ ID NO: 30347 - protein, 9 aa, synthetic construct
GGAGDDWMK

SEQ ID NO: 30348 - protein, 9 aa, synthetic construct
GGAGDDVFP

SEQ ID NO: 30349 - protein, 9 aa, synthetic construct
GGAGDDVFG

SEQ ID NO: 30350 - protein, 9 aa, synthetic construct
GGAGDDWMS

SEQ ID NO: 30351 - protein, 9 aa, synthetic construct
GGAGDDVFE

SEQ ID NO: 30352 - protein, 9 aa, synthetic construct
GGAGDDSVV

SEQ ID NO: 30353 - protein, 9 aa, synthetic construct
GGAGDDSYG

SEQ ID NO: 30354 - protein, 9 aa, synthetic construct
GGAGDDSYI

SEQ ID NO: 30355 - protein, 9 aa, synthetic construct
GGAGDDSYW

SEQ ID NO: 30356 - protein, 9 aa, synthetic construct
GGAGDDTAE

SEQ ID NO: 30357 - protein, 9 aa, synthetic construct
GGAGDDTAF

SEQ ID NO: 30358 - protein, 9 aa, synthetic construct
GGAGDDTAR

SEQ ID NO: 30359 - protein, 9 aa, synthetic construct
GGAGDDTAY

SEQ ID NO: 30360 - protein, 9 aa, synthetic construct
GGAGDDTFE

SEQ ID NO: 30361 - protein, 9 aa, synthetic construct
GGAGDDTFH

SEQ ID NO: 30362 - protein, 9 aa, synthetic construct
GGAGDDTIC

SEQ ID NO: 30363 - protein, 9 aa, synthetic construct
GGAGDDTLC

SEQ ID NO: 30364 - protein, 9 aa, synthetic construct
GGAGDDTVK

SEQ ID NO: 30365 - protein, 9 aa, synthetic construct
GGAGDDTVM

SEQ ID NO: 30366 - protein, 9 aa, synthetic construct
GGAGDDTYA

SEQ ID NO: 30367 - protein, 9 aa, synthetic construct
GGAGDDVAA

SEQ ID NO: 30368 - protein, 9 aa, synthetic construct
GGAGDDVAV

SEQ ID NO: 30369 - protein, 9 aa, synthetic construct
GGAGDDWMM

SEQ ID NO: 30370 - protein, 9 aa, synthetic construct
GGAGDDWVD

SEQ ID NO: 30371 - protein, 9 aa, synthetic construct
GGAGEDFLL

SEQ ID NO: 30372 - protein, 9 aa, synthetic construct
GGAGEDALD

SEQ ID NO: 30373 - protein, 9 aa, synthetic construct
GGAGEDALS

SEQ ID NO: 30374 - protein, 9 aa, synthetic construct
GGAGEDALY

SEQ ID NO: 30375 - protein, 9 aa, synthetic construct
GGAGEDAVF

SEQ ID NO: 30376 - protein, 9 aa, synthetic construct
GGAGEDDIR

SEQ ID NO: 30377 - protein, 9 aa, synthetic construct
GGAGEDDLF

SEQ ID NO: 30378 - protein, 9 aa, synthetic construct
GGAGEDDVD

SEQ ID NO: 30379 - protein, 9 aa, synthetic construct
GGAGEDEAA

SEQ ID NO: 30380 - protein, 9 aa, synthetic construct
GGAGEDEID

SEQ ID NO: 30381 - protein, 9 aa, synthetic construct
GGAGEDEIS

SEQ ID NO: 30382 - protein, 9 aa, synthetic construct
GGAGEDEIV

SEQ ID NO: 30383 - protein, 9 aa, synthetic construct
GGAGEDELE

SEQ ID NO: 30384 - protein, 9 aa, synthetic construct
GGAGEDELG

SEQ ID NO: 30385 - protein, 9 aa, synthetic construct
GGAGEDELQ

SEQ ID NO: 30386 - protein, 9 aa, synthetic construct
GGAGEDELW

SEQ ID NO: 30387 - protein, 9 aa, synthetic construct
GGAGEDEVE

SEQ ID NO: 30388 - protein, 9 aa, synthetic construct
GGAGEDFIS

SEQ ID NO: 30389 - protein, 9 aa, synthetic construct
GGAGEDFLA

SEQ ID NO: 30390 - protein, 9 aa, synthetic construct
GGAGEDALR

SEQ ID NO: 30391 - protein, 9 aa, synthetic construct
GGAGEDAIT

SEQ ID NO: 30392 - protein, 9 aa, synthetic construct
GGAGDDWVG

SEQ ID NO: 30393 - protein, 9 aa, synthetic construct
GGAGEDAIG

SEQ ID NO: 30394 - protein, 9 aa, synthetic construct
GGAGDDWVL

SEQ ID NO: 30395 - protein, 9 aa, synthetic construct
GGAGDDWVR

SEQ ID NO: 30396 - protein, 9 aa, synthetic construct
GGAGDDWVT

SEQ ID NO: 30397 - protein, 9 aa, synthetic construct
GGAGDDWYY

SEQ ID NO: 30398 - protein, 9 aa, synthetic construct
GGAGDDXLF

SEQ ID NO: 30399 - protein, 9 aa, synthetic construct
GGAGDDYAH

SEQ ID NO: 30400 - protein, 9 aa, synthetic construct
GGAGDDYAQ

SEQ ID NO: 30401 - protein, 9 aa, synthetic construct
GGAGDDYFV

SEQ ID NO: 30402 - protein, 9 aa, synthetic construct
GGAGDDYIL

SEQ ID NO: 30403 - protein, 9 aa, synthetic construct
GGAGDDYIR

SEQ ID NO: 30404 - protein, 9 aa, synthetic construct
GGAGDDYMH

SEQ ID NO: 30405 - protein, 9 aa, synthetic construct
GGAGDDYMI

SEQ ID NO: 30406 - protein, 9 aa, synthetic construct
GGAGDDYMS

SEQ ID NO: 30407 - protein, 9 aa, synthetic construct
GGAGDDYMV

SEQ ID NO: 30408 - protein, 9 aa, synthetic construct
GGAGDDYVY

SEQ ID NO: 30409 - protein, 9 aa, synthetic construct
GGAGEDAFN

SEQ ID NO: 30410 - protein, 9 aa, synthetic construct
GGAGEDAFV

SEQ ID NO: 30411 - protein, 9 aa, synthetic construct
GGAGDDGIY

SEQ ID NO: 30412 - protein, 9 aa, synthetic construct
GGAGDDGIW

SEQ ID NO: 30413 - protein, 9 aa, synthetic construct
GGAGDDGIT

SEQ ID NO: 30414 - protein, 9 aa, synthetic construct
GGAGADLIE

SEQ ID NO: 30415 - protein, 9 aa, synthetic construct
GGAGADKIS

SEQ ID NO: 30416 - protein, 9 aa, synthetic construct
GGAGADKLQ

SEQ ID NO: 30417 - protein, 9 aa, synthetic construct
GGAGADKMD

SEQ ID NO: 30418 - protein, 9 aa, synthetic construct
GGAGADKVD

SEQ ID NO: 30419 - protein, 9 aa, synthetic construct
GGAGADKVL

SEQ ID NO: 30420 - protein, 9 aa, synthetic construct
GGAGADKYY

SEQ ID NO: 30421 - protein, 9 aa, synthetic construct
GGAGADLAR

SEQ ID NO: 30422 - protein, 9 aa, synthetic construct
GGAGADLFQ

SEQ ID NO: 30423 - protein, 9 aa, synthetic construct
GGAGADLIH

SEQ ID NO: 30424 - protein, 9 aa, synthetic construct
GGAGDDGIG

SEQ ID NO: 30425 - protein, 9 aa, synthetic construct
GGAGADLIQ

SEQ ID NO: 30426 - protein, 9 aa, synthetic construct
GGAGADLIV

SEQ ID NO: 30427 - protein, 9 aa, synthetic construct
GGAGADLIW

SEQ ID NO: 30428 - protein, 9 aa, synthetic construct
GGAGADLLW

SEQ ID NO: 30429 - protein, 9 aa, synthetic construct
GGAGADLMH

SEQ ID NO: 30430 - protein, 9 aa, synthetic construct
GGAGADLMK

SEQ ID NO: 30431 - protein, 9 aa, synthetic construct
GGAGADLML

SEQ ID NO: 30432 - protein, 9 aa, synthetic construct
GGAGADLMM

SEQ ID NO: 30433 - protein, 9 aa, synthetic construct
GGAGADKIL

SEQ ID NO: 30434 - protein, 9 aa, synthetic construct
GGAGADIYY

SEQ ID NO: 30435 - protein, 9 aa, synthetic construct
GGAGADIYR

SEQ ID NO: 30436 - protein, 9 aa, synthetic construct
GGAGADIVV

SEQ ID NO: 30437 - protein, 9 aa, synthetic construct
GGAGADHIT

SEQ ID NO: 30438 - protein, 9 aa, synthetic construct
GGAGADHLW

SEQ ID NO: 30439 - protein, 9 aa, synthetic construct
GGAGADHMA

SEQ ID NO: 30440 - protein, 9 aa, synthetic construct
GGAGADHMI

SEQ ID NO: 30441 - protein, 9 aa, synthetic construct
GGAGADHMK

SEQ ID NO: 30442 - protein, 9 aa, synthetic construct
GGAGADHML

SEQ ID NO: 30443 - protein, 9 aa, synthetic construct
GGAGADIAE

SEQ ID NO: 30444 - protein, 9 aa, synthetic construct
GGAGADIAR

SEQ ID NO: 30445 - protein, 9 aa, synthetic construct
GGAGADIAY

SEQ ID NO: 30446 - protein, 9 aa, synthetic construct
GGAGADIFI

SEQ ID NO: 30447 - protein, 9 aa, synthetic construct
GGAGADIFY

SEQ ID NO: 30448 - protein, 9 aa, synthetic construct
GGAGADIIM

SEQ ID NO: 30449 - protein, 9 aa, synthetic construct
GGAGADILC

SEQ ID NO: 30450 - protein, 9 aa, synthetic construct
GGAGADILW

SEQ ID NO: 30451 - protein, 9 aa, synthetic construct
GGAGADIMF

SEQ ID NO: 30452 - protein, 9 aa, synthetic construct
GGAGADIMK

SEQ ID NO: 30453 - protein, 9 aa, synthetic construct
GGAGADIVR

SEQ ID NO: 30454 - protein, 9 aa, synthetic construct
GGAGADLMW

SEQ ID NO: 30455 - protein, 9 aa, synthetic construct
GGAGADLYW

SEQ ID NO: 30456 - protein, 9 aa, synthetic construct
GGAGADMAT

SEQ ID NO: 30457 - protein, 9 aa, synthetic construct
GGAGADNMS

SEQ ID NO: 30458 - protein, 9 aa, synthetic construct
GGAGADQFA

SEQ ID NO: 30459 - protein, 9 aa, synthetic construct
GGAGADQFK

SEQ ID NO: 30460 - protein, 9 aa, synthetic construct
GGAGADQFS

SEQ ID NO: 30461 - protein, 9 aa, synthetic construct
GGAGADQFT

SEQ ID NO: 30462 - protein, 9 aa, synthetic construct
GGAGADQFW

SEQ ID NO: 30463 - protein, 9 aa, synthetic construct
GGAGADQID

SEQ ID NO: 30464 - protein, 9 aa, synthetic construct
GGAGADQIL

SEQ ID NO: 30465 - protein, 9 aa, synthetic construct
GGAGADQIN

SEQ ID NO: 30466 - protein, 9 aa, synthetic construct
GGAGADQIQ

SEQ ID NO: 30467 - protein, 9 aa, synthetic construct
GGAGADQMD

SEQ ID NO: 30468 - protein, 9 aa, synthetic construct
GGAGADQME

SEQ ID NO: 30469 - protein, 9 aa, synthetic construct
GGAGADQMS

SEQ ID NO: 30470 - protein, 9 aa, synthetic construct
GGAGADQMY

SEQ ID NO: 30471 - protein, 9 aa, synthetic construct
GGAGADQVF

SEQ ID NO: 30472 - protein, 9 aa, synthetic construct
GGAGADQVG

SEQ ID NO: 30473 - protein, 9 aa, synthetic construct
GGAGADQVI

SEQ ID NO: 30474 - protein, 9 aa, synthetic construct
GGAGADQVQ

SEQ ID NO: 30475 - protein, 9 aa, synthetic construct
GGAGADNVF

SEQ ID NO: 30476 - protein, 9 aa, synthetic construct
GGAGADNMR

SEQ ID NO: 30477 - protein, 9 aa, synthetic construct
GGAGADMFR

SEQ ID NO: 30478 - protein, 9 aa, synthetic construct
GGAGADNMN

SEQ ID NO: 30479 - protein, 9 aa, synthetic construct
GGAGADMFT

SEQ ID NO: 30480 - protein, 9 aa, synthetic construct
GGAGADMIF

SEQ ID NO: 30481 - protein, 9 aa, synthetic construct
GGAGADMIG

SEQ ID NO: 30482 - protein, 9 aa, synthetic construct
GGAGADMIS

SEQ ID NO: 30483 - protein, 9 aa, synthetic construct
GGAGADMLK

SEQ ID NO: 30484 - protein, 9 aa, synthetic construct
GGAGADMLQ

SEQ ID NO: 30485 - protein, 9 aa, synthetic construct
GGAGADMMD

SEQ ID NO: 30486 - protein, 9 aa, synthetic construct
GGAGADMMK

SEQ ID NO: 30487 - protein, 9 aa, synthetic construct
GGAGADMMW

SEQ ID NO: 30488 - protein, 9 aa, synthetic construct
GGAGADMVF

SEQ ID NO: 30489 - protein, 9 aa, synthetic construct
GGAGADNAV

SEQ ID NO: 30490 - protein, 9 aa, synthetic construct
GGAGADNFI

SEQ ID NO: 30491 - protein, 9 aa, synthetic construct
GGAGADNII

SEQ ID NO: 30492 - protein, 9 aa, synthetic construct
GGAGADNIQ

SEQ ID NO: 30493 - protein, 9 aa, synthetic construct
GGAGADNLK

SEQ ID NO: 30494 - protein, 9 aa, synthetic construct
GGAGADNLR

SEQ ID NO: 30495 - protein, 9 aa, synthetic construct
GGAGADNMK

SEQ ID NO: 30496 - protein, 9 aa, synthetic construct
GGAGADHIK

SEQ ID NO: 30497 - protein, 9 aa, synthetic construct
GGAGADHFR

SEQ ID NO: 30498 - protein, 9 aa, synthetic construct
GGAGADHFK

SEQ ID NO: 30499 - protein, 9 aa, synthetic construct
GGAGADDIK

SEQ ID NO: 30500 - protein, 9 aa, synthetic construct
GGAGADDIS

SEQ ID NO: 30501 - protein, 9 aa, synthetic construct
GGAGADDIY

SEQ ID NO: 30502 - protein, 9 aa, synthetic construct
GGAGADDLK

SEQ ID NO: 30503 - protein, 9 aa, synthetic construct
GGAGADDMA

SEQ ID NO: 30504 - protein, 9 aa, synthetic construct
GGAGADEAS

SEQ ID NO: 30505 - protein, 9 aa, synthetic construct
GGAGADEAY

SEQ ID NO: 30506 - protein, 9 aa, synthetic construct
GGAGADEFF

SEQ ID NO: 30507 - protein, 9 aa, synthetic construct
GGAGADEFI

SEQ ID NO: 30508 - protein, 9 aa, synthetic construct
GGAGADEFQ

SEQ ID NO: 30509 - protein, 9 aa, synthetic construct
GGAGADEIE

SEQ ID NO: 30510 - protein, 9 aa, synthetic construct
GGAGADEIF

SEQ ID NO: 30511 - protein, 9 aa, synthetic construct
GGAGADEIH

SEQ ID NO: 30512 - protein, 9 aa, synthetic construct
GGAGADEIN

SEQ ID NO: 30513 - protein, 9 aa, synthetic construct
GGAGADEIQ

SEQ ID NO: 30514 - protein, 9 aa, synthetic construct
GGAGADELH

SEQ ID NO: 30515 - protein, 9 aa, synthetic construct
GGAGADELK

SEQ ID NO: 30516 - protein, 9 aa, synthetic construct
GGAGADEMF

SEQ ID NO: 30517 - protein, 9 aa, synthetic construct
GGAGADDIN

SEQ ID NO: 30518 - protein, 9 aa, synthetic construct
GGAGADDIF

SEQ ID NO: 30519 - protein, 9 aa, synthetic construct
GGAGADEVI

SEQ ID NO: 30520 - protein, 9 aa, synthetic construct
GGAGADDFL

SEQ ID NO: 30521 - protein, 9 aa, synthetic construct
GGAGADAFA

SEQ ID NO: 30522 - protein, 9 aa, synthetic construct
GGAGADAFK

SEQ ID NO: 30523 - protein, 9 aa, synthetic construct
GGAGADAFM

SEQ ID NO: 30524 - protein, 9 aa, synthetic construct
GGAGADAFN

SEQ ID NO: 30525 - protein, 9 aa, synthetic construct
GGAGADAIG

SEQ ID NO: 30526 - protein, 9 aa, synthetic construct
GGAGADAIS

SEQ ID NO: 30527 - protein, 9 aa, synthetic construct
GGAGADALG

SEQ ID NO: 30528 - protein, 9 aa, synthetic construct
GGAGADAMK

SEQ ID NO: 30529 - protein, 9 aa, synthetic construct
GGAGADAMR

SEQ ID NO: 30530 - protein, 9 aa, synthetic construct
GGAGADAVG

SEQ ID NO: 30531 - protein, 9 aa, synthetic construct
GGAGADAVH

SEQ ID NO: 30532 - protein, 9 aa, synthetic construct
GGAGADAYI

SEQ ID NO: 30533 - protein, 9 aa, synthetic construct
GGAGADCFI

SEQ ID NO: 30534 - protein, 9 aa, synthetic construct
GGAGADCVG

SEQ ID NO: 30535 - protein, 9 aa, synthetic construct
GGAGADCYV

SEQ ID NO: 30536 - protein, 9 aa, synthetic construct
GGAGADDFF

SEQ ID NO: 30537 - protein, 9 aa, synthetic construct
GGAGADDFH

SEQ ID NO: 30538 - protein, 9 aa, synthetic construct
GGAGADEMV

SEQ ID NO: 30539 - protein, 9 aa, synthetic construct
GGAGADEVR

SEQ ID NO: 30540 - protein, 9 aa, synthetic construct
GGAGADHFG

SEQ ID NO: 30541 - protein, 9 aa, synthetic construct
GGAGADFMQ

SEQ ID NO: 30542 - protein, 9 aa, synthetic construct
GGAGADFMV

SEQ ID NO: 30543 - protein, 9 aa, synthetic construct
GGAGADFMY

SEQ ID NO: 30544 - protein, 9 aa, synthetic construct
GGAGADFVL

SEQ ID NO: 30545 - protein, 9 aa, synthetic construct
GGAGADFVT

SEQ ID NO: 30546 - protein, 9 aa, synthetic construct
GGAGADFVY

SEQ ID NO: 30547 - protein, 9 aa, synthetic construct
GGAGADGFI

SEQ ID NO: 30548 - protein, 9 aa, synthetic construct
GGAGADGFV

SEQ ID NO: 30549 - protein, 9 aa, synthetic construct
GGAGADGIL

SEQ ID NO: 30550 - protein, 9 aa, synthetic construct
GGAGADGLN

SEQ ID NO: 30551 - protein, 9 aa, synthetic construct
GGAGADGLT

SEQ ID NO: 30552 - protein, 9 aa, synthetic construct
GGAGADGMF

SEQ ID NO: 30553 - protein, 9 aa, synthetic construct
GGAGADGMH

SEQ ID NO: 30554 - protein, 9 aa, synthetic construct
GGAGADGMS

SEQ ID NO: 30555 - protein, 9 aa, synthetic construct
GGAGADGMT

SEQ ID NO: 30556 - protein, 9 aa, synthetic construct
GGAGADGVS

SEQ ID NO: 30557 - protein, 9 aa, synthetic construct
GGAGADHFD

SEQ ID NO: 30558 - protein, 9 aa, synthetic construct
GGAGADHFF

SEQ ID NO: 30559 - protein, 9 aa, synthetic construct
GGAGADFMS

SEQ ID NO: 30560 - protein, 9 aa, synthetic construct
GGAGADFMN

SEQ ID NO: 30561 - protein, 9 aa, synthetic construct
GGAGADEVS

SEQ ID NO: 30562 - protein, 9 aa, synthetic construct
GGAGADFML

SEQ ID NO: 30563 - protein, 9 aa, synthetic construct
GGAGADFAL

SEQ ID NO: 30564 - protein, 9 aa, synthetic construct
GGAGADFAM

SEQ ID NO: 30565 - protein, 9 aa, synthetic construct
GGAGADFAQ

SEQ ID NO: 30566 - protein, 9 aa, synthetic construct
GGAGADFAR

SEQ ID NO: 30567 - protein, 9 aa, synthetic construct
GGAGADFAS

SEQ ID NO: 30568 - protein, 9 aa, synthetic construct
GGAGADFFI

SEQ ID NO: 30569 - protein, 9 aa, synthetic construct
GGAGADFFN

SEQ ID NO: 30570 - protein, 9 aa, synthetic construct
GGAGADFFR

SEQ ID NO: 30571 - protein, 9 aa, synthetic construct
GGAGADFFT

SEQ ID NO: 30572 - protein, 9 aa, synthetic construct
GGAGADFIS

SEQ ID NO: 30573 - protein, 9 aa, synthetic construct
GGAGADFLE

SEQ ID NO: 30574 - protein, 9 aa, synthetic construct
GGAGADFLG

SEQ ID NO: 30575 - protein, 9 aa, synthetic construct
GGAGADFLH

SEQ ID NO: 30576 - protein, 9 aa, synthetic construct
GGAGADFLL

SEQ ID NO: 30577 - protein, 9 aa, synthetic construct
GGAGADFLQ

SEQ ID NO: 30578 - protein, 9 aa, synthetic construct
GGAGADFME

SEQ ID NO: 30579 - protein, 9 aa, synthetic construct
GGAGADFMK

SEQ ID NO: 30580 - protein, 9 aa, synthetic construct
GGAGADQVY

SEQ ID NO: 30581 - protein, 9 aa, synthetic construct
GGAGADRFD

SEQ ID NO: 30582 - protein, 9 aa, synthetic construct
GGAGADRFN

SEQ ID NO: 30583 - protein, 9 aa, synthetic construct
GGAGDDAVI

SEQ ID NO: 30584 - protein, 9 aa, synthetic construct
GGAGDDAYI

SEQ ID NO: 30585 - protein, 9 aa, synthetic construct
GGAGDDCIA

SEQ ID NO: 30586 - protein, 9 aa, synthetic construct
GGAGDDCIR

SEQ ID NO: 30587 - protein, 9 aa, synthetic construct
GGAGDDCLI

SEQ ID NO: 30588 - protein, 9 aa, synthetic construct
GGAGDDCLT

SEQ ID NO: 30589 - protein, 9 aa, synthetic construct
GGAGDDDIL

SEQ ID NO: 30590 - protein, 9 aa, synthetic construct
GGAGDDDIQ

SEQ ID NO: 30591 - protein, 9 aa, synthetic construct
GGAGDDDIY

SEQ ID NO: 30592 - protein, 9 aa, synthetic construct
GGAGDDDLA

SEQ ID NO: 30593 - protein, 9 aa, synthetic construct
GGAGDDDLE

SEQ ID NO: 30594 - protein, 9 aa, synthetic construct
GGAGDDDLG

SEQ ID NO: 30595 - protein, 9 aa, synthetic construct
GGAGDDDLN

SEQ ID NO: 30596 - protein, 9 aa, synthetic construct
GGAGDDDMV

SEQ ID NO: 30597 - protein, 9 aa, synthetic construct
GGAGDDDMY

SEQ ID NO: 30598 - protein, 9 aa, synthetic construct
GGAGDDDVA

SEQ ID NO: 30599 - protein, 9 aa, synthetic construct
GGAGDDDVF

SEQ ID NO: 30600 - protein, 9 aa, synthetic construct
GGAGDDDYF

SEQ ID NO: 30601 - protein, 9 aa, synthetic construct
GGAGDDAVL

SEQ ID NO: 30602 - protein, 9 aa, synthetic construct
GGAGDDAVH

SEQ ID NO: 30603 - protein, 9 aa, synthetic construct
GGAGDDEAH

SEQ ID NO: 30604 - protein, 9 aa, synthetic construct
GGAGDDAVF

SEQ ID NO: 30605 - protein, 9 aa, synthetic construct
GGAGCDSLY

SEQ ID NO: 30606 - protein, 9 aa, synthetic construct
GGAGCDTLA

SEQ ID NO: 30607 - protein, 9 aa, synthetic construct
GGAGCDTLV

SEQ ID NO: 30608 - protein, 9 aa, synthetic construct
GGAGCDVLN

SEQ ID NO: 30609 - protein, 9 aa, synthetic construct
GGAGCDWIE

SEQ ID NO: 30610 - protein, 9 aa, synthetic construct
GGAGDDAAS

SEQ ID NO: 30611 - protein, 9 aa, synthetic construct
GGAGDDAAV

SEQ ID NO: 30612 - protein, 9 aa, synthetic construct
GGAGDDAFA

SEQ ID NO: 30613 - protein, 9 aa, synthetic construct
GGAGDDAFG

SEQ ID NO: 30614 - protein, 9 aa, synthetic construct
GGAGDDAFV

SEQ ID NO: 30615 - protein, 9 aa, synthetic construct
GGAGDDAFY

SEQ ID NO: 30616 - protein, 9 aa, synthetic construct
GGAGDDAIK

SEQ ID NO: 30617 - protein, 9 aa, synthetic construct
GGAGDDAIQ

SEQ ID NO: 30618 - protein, 9 aa, synthetic construct
GGAGDDAIR

SEQ ID NO: 30619 - protein, 9 aa, synthetic construct
GGAGDDAIV

SEQ ID NO: 30620 - protein, 9 aa, synthetic construct
GGAGDDAMS

SEQ ID NO: 30621 - protein, 9 aa, synthetic construct
GGAGDDAMV

SEQ ID NO: 30622 - protein, 9 aa, synthetic construct
GGAGDDEAG

SEQ ID NO: 30623 - protein, 9 aa, synthetic construct
GGAGDDEAR

SEQ ID NO: 30624 - protein, 9 aa, synthetic construct
GGAGCDLLI

SEQ ID NO: 30625 - protein, 9 aa, synthetic construct
GGAGDDEYL

SEQ ID NO: 30626 - protein, 9 aa, synthetic construct
GGAGDDFAY

SEQ ID NO: 30627 - protein, 9 aa, synthetic construct
GGAGDDFFV

SEQ ID NO: 30628 - protein, 9 aa, synthetic construct
GGAGDDFIW

SEQ ID NO: 30629 - protein, 9 aa, synthetic construct
GGAGDDFMA

SEQ ID NO: 30630 - protein, 9 aa, synthetic construct
GGAGDDFMD

SEQ ID NO: 30631 - protein, 9 aa, synthetic construct
GGAGDDFME

SEQ ID NO: 30632 - protein, 9 aa, synthetic construct
GGAGDDFMR

SEQ ID NO: 30633 - protein, 9 aa, synthetic construct
GGAGDDFVD

SEQ ID NO: 30634 - protein, 9 aa, synthetic construct
GGAGDDFVF

SEQ ID NO: 30635 - protein, 9 aa, synthetic construct
GGAGDDFVI

SEQ ID NO: 30636 - protein, 9 aa, synthetic construct
GGAGDDFVQ

SEQ ID NO: 30637 - protein, 9 aa, synthetic construct
GGAGDDFVS

SEQ ID NO: 30638 - protein, 9 aa, synthetic construct
GGAGDDFYT

SEQ ID NO: 30639 - protein, 9 aa, synthetic construct
GGAGDDFYY

SEQ ID NO: 30640 - protein, 9 aa, synthetic construct
GGAGDDGAT

SEQ ID NO: 30641 - protein, 9 aa, synthetic construct
GGAGDDGAV

SEQ ID NO: 30642 - protein, 9 aa, synthetic construct
GGAGDDGFI

SEQ ID NO: 30643 - protein, 9 aa, synthetic construct
GGAGDDFAE

SEQ ID NO: 30644 - protein, 9 aa, synthetic construct
GGAGDDEYI

SEQ ID NO: 30645 - protein, 9 aa, synthetic construct
GGAGDDEFD

SEQ ID NO: 30646 - protein, 9 aa, synthetic construct
GGAGDDEVT

SEQ ID NO: 30647 - protein, 9 aa, synthetic construct
GGAGDDEFI

SEQ ID NO: 30648 - protein, 9 aa, synthetic construct
GGAGDDEFT

SEQ ID NO: 30649 - protein, 9 aa, synthetic construct
GGAGDDEIG

SEQ ID NO: 30650 - protein, 9 aa, synthetic construct
GGAGDDEIN

SEQ ID NO: 30651 - protein, 9 aa, synthetic construct
GGAGDDELC

SEQ ID NO: 30652 - protein, 9 aa, synthetic construct
GGAGDDELM

SEQ ID NO: 30653 - protein, 9 aa, synthetic construct
GGAGDDEMD

SEQ ID NO: 30654 - protein, 9 aa, synthetic construct
GGAGDDEML

SEQ ID NO: 30655 - protein, 9 aa, synthetic construct
GGAGDDEMV

SEQ ID NO: 30656 - protein, 9 aa, synthetic construct
GGAGDDEMY

SEQ ID NO: 30657 - protein, 9 aa, synthetic construct
GGAGDDEVA

SEQ ID NO: 30658 - protein, 9 aa, synthetic construct
GGAGDDEVF

SEQ ID NO: 30659 - protein, 9 aa, synthetic construct
GGAGDDEVG

SEQ ID NO: 30660 - protein, 9 aa, synthetic construct
GGAGDDEVK

SEQ ID NO: 30661 - protein, 9 aa, synthetic construct
GGAGDDEVL

SEQ ID NO: 30662 - protein, 9 aa, synthetic construct
GGAGDDEVN

SEQ ID NO: 30663 - protein, 9 aa, synthetic construct
GGAGDDEVS

SEQ ID NO: 30664 - protein, 9 aa, synthetic construct
GGAGCDRVR

SEQ ID NO: 30665 - protein, 9 aa, synthetic construct
GGAGCDDIL

SEQ ID NO: 30666 - protein, 9 aa, synthetic construct
GGAGADRFT

SEQ ID NO: 30667 - protein, 9 aa, synthetic construct
GGAGADSVS

SEQ ID NO: 30668 - protein, 9 aa, synthetic construct
GGAGADTAE

SEQ ID NO: 30669 - protein, 9 aa, synthetic construct
GGAGADTAQ

SEQ ID NO: 30670 - protein, 9 aa, synthetic construct
GGAGADTAY

SEQ ID NO: 30671 - protein, 9 aa, synthetic construct
GGAGADTIM

SEQ ID NO: 30672 - protein, 9 aa, synthetic construct
GGAGADTIW

SEQ ID NO: 30673 - protein, 9 aa, synthetic construct
GGAGADTLC

SEQ ID NO: 30674 - protein, 9 aa, synthetic construct
GGAGADTMM

SEQ ID NO: 30675 - protein, 9 aa, synthetic construct
GGAGADTVK

SEQ ID NO: 30676 - protein, 9 aa, synthetic construct
GGAGADTYE

SEQ ID NO: 30677 - protein, 9 aa, synthetic construct
GGAGADTYF

SEQ ID NO: 30678 - protein, 9 aa, synthetic construct
GGAGADTYG

SEQ ID NO: 30679 - protein, 9 aa, synthetic construct
GGAGADTYN

SEQ ID NO: 30680 - protein, 9 aa, synthetic construct
GGAGADVAG

SEQ ID NO: 30681 - protein, 9 aa, synthetic construct
GGAGADVFG

SEQ ID NO: 30682 - protein, 9 aa, synthetic construct
GGAGADVFM

SEQ ID NO: 30683 - protein, 9 aa, synthetic construct
GGAGADVFT

SEQ ID NO: 30684 - protein, 9 aa, synthetic construct
GGAGADVIF

SEQ ID NO: 30685 - protein, 9 aa, synthetic construct
GGAGADSVT

SEQ ID NO: 30686 - protein, 9 aa, synthetic construct
GGAGADSVI

SEQ ID NO: 30687 - protein, 9 aa, synthetic construct
GGAGADVMQ

SEQ ID NO: 30688 - protein, 9 aa, synthetic construct
GGAGADSMR

SEQ ID NO: 30689 - protein, 9 aa, synthetic construct
GGAGADRFW

SEQ ID NO: 30690 - protein, 9 aa, synthetic construct
GGAGADRIK

SEQ ID NO: 30691 - protein, 9 aa, synthetic construct
GGAGADRIW

SEQ ID NO: 30692 - protein, 9 aa, synthetic construct
GGAGADRMK

SEQ ID NO: 30693 - protein, 9 aa, synthetic construct
GGAGADRMN

SEQ ID NO: 30694 - protein, 9 aa, synthetic construct
GGAGADRVD

SEQ ID NO: 30695 - protein, 9 aa, synthetic construct
GGAGADRVL

SEQ ID NO: 30696 - protein, 9 aa, synthetic construct
GGAGADRVW

SEQ ID NO: 30697 - protein, 9 aa, synthetic construct
GGAGADRVY

SEQ ID NO: 30698 - protein, 9 aa, synthetic construct
GGAGADRYI

SEQ ID NO: 30699 - protein, 9 aa, synthetic construct
GGAGADRYS

SEQ ID NO: 30700 - protein, 9 aa, synthetic construct
GGAGADSFF

SEQ ID NO: 30701 - protein, 9 aa, synthetic construct
GGAGADSFM

SEQ ID NO: 30702 - protein, 9 aa, synthetic construct
GGAGADSFQ

SEQ ID NO: 30703 - protein, 9 aa, synthetic construct
GGAGADSFS

SEQ ID NO: 30704 - protein, 9 aa, synthetic construct
GGAGADSFW

SEQ ID NO: 30705 - protein, 9 aa, synthetic construct
GGAGADSFY

SEQ ID NO: 30706 - protein, 9 aa, synthetic construct
GGAGADVIG

SEQ ID NO: 30707 - protein, 9 aa, synthetic construct
GGAGADVVA

SEQ ID NO: 30708 - protein, 9 aa, synthetic construct
GGAGCDALS

SEQ ID NO: 30709 - protein, 9 aa, synthetic construct
GGAGADWMQ

SEQ ID NO: 30710 - protein, 9 aa, synthetic construct
GGAGADWVD

SEQ ID NO: 30711 - protein, 9 aa, synthetic construct
GGAGADWVV

SEQ ID NO: 30712 - protein, 9 aa, synthetic construct
GGAGADWYW

SEQ ID NO: 30713 - protein, 9 aa, synthetic construct
GGAGADXIT

SEQ ID NO: 30714 - protein, 9 aa, synthetic construct
GGAGADXIV

SEQ ID NO: 30715 - protein, 9 aa, synthetic construct
GGAGADXVK

SEQ ID NO: 30716 - protein, 9 aa, synthetic construct
GGAGADYAD

SEQ ID NO: 30717 - protein, 9 aa, synthetic construct
GGAGADYFA

SEQ ID NO: 30718 - protein, 9 aa, synthetic construct
GGAGADYFG

SEQ ID NO: 30719 - protein, 9 aa, synthetic construct
GGAGADYFI

SEQ ID NO: 30720 - protein, 9 aa, synthetic construct
GGAGADYFQ

SEQ ID NO: 30721 - protein, 9 aa, synthetic construct
GGAGADYLI

SEQ ID NO: 30722 - protein, 9 aa, synthetic construct
GGAGADYMS

SEQ ID NO: 30723 - protein, 9 aa, synthetic construct
GGAGADYMY

SEQ ID NO: 30724 - protein, 9 aa, synthetic construct
GGAGADYVA

SEQ ID NO: 30725 - protein, 9 aa, synthetic construct
GGAGADYVV

SEQ ID NO: 30726 - protein, 9 aa, synthetic construct
GGAGADYVY

SEQ ID NO: 30727 - protein, 9 aa, synthetic construct
GGAGADWVA

SEQ ID NO: 30728 - protein, 9 aa, synthetic construct
GGAGADWMH

SEQ ID NO: 30729 - protein, 9 aa, synthetic construct
GGAGADVVF

SEQ ID NO: 30730 - protein, 9 aa, synthetic construct
GGAGADWME

SEQ ID NO: 30731 - protein, 9 aa, synthetic construct
GGAGADVVI

SEQ ID NO: 30732 - protein, 9 aa, synthetic construct
GGAGADVVL

SEQ ID NO: 30733 - protein, 9 aa, synthetic construct
GGAGADVVR

SEQ ID NO: 30734 - protein, 9 aa, synthetic construct
GGAGADVVT

SEQ ID NO: 30735 - protein, 9 aa, synthetic construct
GGAGADVYI

SEQ ID NO: 30736 - protein, 9 aa, synthetic construct
GGAGADVYM

SEQ ID NO: 30737 - protein, 9 aa, synthetic construct
GGAGADVYY

SEQ ID NO: 30738 - protein, 9 aa, synthetic construct
GGAGADWFI

SEQ ID NO: 30739 - protein, 9 aa, synthetic construct
GGAGADWFV

SEQ ID NO: 30740 - protein, 9 aa, synthetic construct
GGAGADWIE

SEQ ID NO: 30741 - protein, 9 aa, synthetic construct
GGAGADWIL

SEQ ID NO: 30742 - protein, 9 aa, synthetic construct
GGAGADWIN

SEQ ID NO: 30743 - protein, 9 aa, synthetic construct
GGAGADWIR

SEQ ID NO: 30744 - protein, 9 aa, synthetic construct
GGAGADWLF

SEQ ID NO: 30745 - protein, 9 aa, synthetic construct
GGAGADWLI

SEQ ID NO: 30746 - protein, 9 aa, synthetic construct
GGAGADWLN

SEQ ID NO: 30747 - protein, 9 aa, synthetic construct
GGAGADWLT

SEQ ID NO: 30748 - protein, 9 aa, synthetic construct
GGAGEDTMR

SEQ ID NO: 30749 - protein, 9 aa, synthetic construct
GGAGEDVAD

SEQ ID NO: 30750 - protein, 9 aa, synthetic construct
GGAGKDIMF

SEQ ID NO: 30751 - protein, 9 aa, synthetic construct
GGAGHDVLY

SEQ ID NO: 30752 - protein, 9 aa, synthetic construct
GGAGHDTYH

SEQ ID NO: 30753 - protein, 9 aa, synthetic construct
GGAGHDTYY

SEQ ID NO: 30754 - protein, 9 aa, synthetic construct
GGAGHDVAY

SEQ ID NO: 30755 - protein, 9 aa, synthetic construct
GGAGHDVFA

SEQ ID NO: 30756 - protein, 9 aa, synthetic construct
GGAGHDVFR

SEQ ID NO: 30757 - protein, 9 aa, synthetic construct
GGAGHDVIE

SEQ ID NO: 30758 - protein, 9 aa, synthetic construct
GGAGHDVIR

SEQ ID NO: 30759 - protein, 9 aa, synthetic construct
GGAGHDVLN

SEQ ID NO: 30760 - protein, 9 aa, synthetic construct
GGAGHDVVY

SEQ ID NO: 30761 - protein, 9 aa, synthetic construct
GGAGIDILD

SEQ ID NO: 30762 - protein, 9 aa, synthetic construct
GGAGHDVYY

SEQ ID NO: 30763 - protein, 9 aa, synthetic construct
GGAGHDWIA

SEQ ID NO: 30764 - protein, 9 aa, synthetic construct
GGAGHDWIN

SEQ ID NO: 30765 - protein, 9 aa, synthetic construct
GGAGHDWIQ

SEQ ID NO: 30766 - protein, 9 aa, synthetic construct
GGAGHDWIW

SEQ ID NO: 30767 - protein, 9 aa, synthetic construct
GGAGHDWLD

SEQ ID NO: 30768 - protein, 9 aa, synthetic construct
GGAGHDWLE

SEQ ID NO: 30769 - protein, 9 aa, synthetic construct
GGAGHDWLF

SEQ ID NO: 30770 - protein, 9 aa, synthetic construct
GGAGHDTVF

SEQ ID NO: 30771 - protein, 9 aa, synthetic construct
GGAGHDTMS

SEQ ID NO: 30772 - protein, 9 aa, synthetic construct
GGAGHDTMI

SEQ ID NO: 30773 - protein, 9 aa, synthetic construct
GGAGHDTMD

SEQ ID NO: 30774 - protein, 9 aa, synthetic construct
GGAGHDSLI

SEQ ID NO: 30775 - protein, 9 aa, synthetic construct
GGAGHDSLN

SEQ ID NO: 30776 - protein, 9 aa, synthetic construct
GGAGHDSLQ

SEQ ID NO: 30777 - protein, 9 aa, synthetic construct
GGAGHDSVD

SEQ ID NO: 30778 - protein, 9 aa, synthetic construct
GGAGHDSYY

SEQ ID NO: 30779 - protein, 9 aa, synthetic construct
GGAGHDTAY

SEQ ID NO: 30780 - protein, 9 aa, synthetic construct
GGAGHDTFD

SEQ ID NO: 30781 - protein, 9 aa, synthetic construct
GGAGHDTFK

SEQ ID NO: 30782 - protein, 9 aa, synthetic construct
GGAGHDTIA

SEQ ID NO: 30783 - protein, 9 aa, synthetic construct
GGAGHDTIF

SEQ ID NO: 30784 - protein, 9 aa, synthetic construct
GGAGHDTIN

SEQ ID NO: 30785 - protein, 9 aa, synthetic construct
GGAGHDTIQ

SEQ ID NO: 30786 - protein, 9 aa, synthetic construct
GGAGHDTIV

SEQ ID NO: 30787 - protein, 9 aa, synthetic construct
GGAGHDTIW

SEQ ID NO: 30788 - protein, 9 aa, synthetic construct
GGAGHDTLC

SEQ ID NO: 30789 - protein, 9 aa, synthetic construct
GGAGHDTLM

SEQ ID NO: 30790 - protein, 9 aa, synthetic construct
GGAGHDTMA

SEQ ID NO: 30791 - protein, 9 aa, synthetic construct
GGAGHDWLK

SEQ ID NO: 30792 - protein, 9 aa, synthetic construct
GGAGHDWLT

SEQ ID NO: 30793 - protein, 9 aa, synthetic construct
GGAGHDWLY

SEQ ID NO: 30794 - protein, 9 aa, synthetic construct
GGAGIDELY

SEQ ID NO: 30795 - protein, 9 aa, synthetic construct
GGAGIDFLD

SEQ ID NO: 30796 - protein, 9 aa, synthetic construct
GGAGIDFLH

SEQ ID NO: 30797 - protein, 9 aa, synthetic construct
GGAGIDFLN

SEQ ID NO: 30798 - protein, 9 aa, synthetic construct
GGAGIDFLS

SEQ ID NO: 30799 - protein, 9 aa, synthetic construct
GGAGIDFLW

SEQ ID NO: 30800 - protein, 9 aa, synthetic construct
GGAGIDFLY

SEQ ID NO: 30801 - protein, 9 aa, synthetic construct
GGAGIDFMY

SEQ ID NO: 30802 - protein, 9 aa, synthetic construct
GGAGIDFVD

SEQ ID NO: 30803 - protein, 9 aa, synthetic construct
GGAGIDFVS

SEQ ID NO: 30804 - protein, 9 aa, synthetic construct
GGAGIDGLS

SEQ ID NO: 30805 - protein, 9 aa, synthetic construct
GGAGIDGVS

SEQ ID NO: 30806 - protein, 9 aa, synthetic construct
GGAGIDHIS

SEQ ID NO: 30807 - protein, 9 aa, synthetic construct
GGAGIDHMF

SEQ ID NO: 30808 - protein, 9 aa, synthetic construct
GGAGIDHMY

SEQ ID NO: 30809 - protein, 9 aa, synthetic construct
GGAGIDIAN

SEQ ID NO: 30810 - protein, 9 aa, synthetic construct
GGAGIDIIS

SEQ ID NO: 30811 - protein, 9 aa, synthetic construct
GGAGIDIIT

SEQ ID NO: 30812 - protein, 9 aa, synthetic construct
GGAGIDFFR

SEQ ID NO: 30813 - protein, 9 aa, synthetic construct
GGAGIDELN

SEQ ID NO: 30814 - protein, 9 aa, synthetic construct
GGAGHDYIE

SEQ ID NO: 30815 - protein, 9 aa, synthetic construct
GGAGIDEID

SEQ ID NO: 30816 - protein, 9 aa, synthetic construct
GGAGHDYVF

SEQ ID NO: 30817 - protein, 9 aa, synthetic construct
GGAGHDYVV

SEQ ID NO: 30818 - protein, 9 aa, synthetic construct
GGAGIDAAV

SEQ ID NO: 30819 - protein, 9 aa, synthetic construct
GGAGIDAIE

SEQ ID NO: 30820 - protein, 9 aa, synthetic construct
GGAGIDALI

SEQ ID NO: 30821 - protein, 9 aa, synthetic construct
GGAGIDALR

SEQ ID NO: 30822 - protein, 9 aa, synthetic construct
GGAGIDALV

SEQ ID NO: 30823 - protein, 9 aa, synthetic construct
GGAGIDAMI

SEQ ID NO: 30824 - protein, 9 aa, synthetic construct
GGAGIDAMQ

SEQ ID NO: 30825 - protein, 9 aa, synthetic construct
GGAGIDAMY

SEQ ID NO: 30826 - protein, 9 aa, synthetic construct
GGAGIDAVW

SEQ ID NO: 30827 - protein, 9 aa, synthetic construct
GGAGIDDIY

SEQ ID NO: 30828 - protein, 9 aa, synthetic construct
GGAGIDDLI

SEQ ID NO: 30829 - protein, 9 aa, synthetic construct
GGAGIDDLS

SEQ ID NO: 30830 - protein, 9 aa, synthetic construct
GGAGIDDLT

SEQ ID NO: 30831 - protein, 9 aa, synthetic construct
GGAGIDDMN

SEQ ID NO: 30832 - protein, 9 aa, synthetic construct
GGAGIDEAD

SEQ ID NO: 30833 - protein, 9 aa, synthetic construct
GGAGHDSLH

SEQ ID NO: 30834 - protein, 9 aa, synthetic construct
GGAGHDSIV

SEQ ID NO: 30835 - protein, 9 aa, synthetic construct
GGAGHDSIR

SEQ ID NO: 30836 - protein, 9 aa, synthetic construct
GGAGHDIIM

SEQ ID NO: 30837 - protein, 9 aa, synthetic construct
GGAGHDIIV

SEQ ID NO: 30838 - protein, 9 aa, synthetic construct
GGAGHDILD

SEQ ID NO: 30839 - protein, 9 aa, synthetic construct
GGAGHDILF

SEQ ID NO: 30840 - protein, 9 aa, synthetic construct
GGAGHDILL

SEQ ID NO: 30841 - protein, 9 aa, synthetic construct
GGAGHDILY

SEQ ID NO: 30842 - protein, 9 aa, synthetic construct
GGAGHDIMF

SEQ ID NO: 30843 - protein, 9 aa, synthetic construct
GGAGHDIVA

SEQ ID NO: 30844 - protein, 9 aa, synthetic construct
GGAGHDIVN

SEQ ID NO: 30845 - protein, 9 aa, synthetic construct
GGAGHDIYI

SEQ ID NO: 30846 - protein, 9 aa, synthetic construct
GGAGHDIYV

SEQ ID NO: 30847 - protein, 9 aa, synthetic construct
GGAGHDKID

SEQ ID NO: 30848 - protein, 9 aa, synthetic construct
GGAGHDKIS

SEQ ID NO: 30849 - protein, 9 aa, synthetic construct
GGAGHDKLF

SEQ ID NO: 30850 - protein, 9 aa, synthetic construct
GGAGHDKLI

SEQ ID NO: 30851 - protein, 9 aa, synthetic construct
GGAGHDKLM

SEQ ID NO: 30852 - protein, 9 aa, synthetic construct
GGAGHDKLW

SEQ ID NO: 30853 - protein, 9 aa, synthetic construct
GGAGHDKLY

SEQ ID NO: 30854 - protein, 9 aa, synthetic construct
GGAGHDIIT

SEQ ID NO: 30855 - protein, 9 aa, synthetic construct
GGAGHDIIK

SEQ ID NO: 30856 - protein, 9 aa, synthetic construct
GGAGHDLIK

SEQ ID NO: 30857 - protein, 9 aa, synthetic construct
GGAGHDIAR

SEQ ID NO: 30858 - protein, 9 aa, synthetic construct
GGAGHDFIN

SEQ ID NO: 30859 - protein, 9 aa, synthetic construct
GGAGHDFIS

SEQ ID NO: 30860 - protein, 9 aa, synthetic construct
GGAGHDFLA

SEQ ID NO: 30861 - protein, 9 aa, synthetic construct
GGAGHDFLI

SEQ ID NO: 30862 - protein, 9 aa, synthetic construct
GGAGHDFLS

SEQ ID NO: 30863 - protein, 9 aa, synthetic construct
GGAGHDFMM

SEQ ID NO: 30864 - protein, 9 aa, synthetic construct
GGAGHDFVS

SEQ ID NO: 30865 - protein, 9 aa, synthetic construct
GGAGHDGIE

SEQ ID NO: 30866 - protein, 9 aa, synthetic construct
GGAGHDGIV

SEQ ID NO: 30867 - protein, 9 aa, synthetic construct
GGAGHDGLI

SEQ ID NO: 30868 - protein, 9 aa, synthetic construct
GGAGHDGLW

SEQ ID NO: 30869 - protein, 9 aa, synthetic construct
GGAGHDHIL

SEQ ID NO: 30870 - protein, 9 aa, synthetic construct
GGAGHDHIS

SEQ ID NO: 30871 - protein, 9 aa, synthetic construct
GGAGHDHLT

SEQ ID NO: 30872 - protein, 9 aa, synthetic construct
GGAGHDHLV

SEQ ID NO: 30873 - protein, 9 aa, synthetic construct
GGAGHDHLY

SEQ ID NO: 30874 - protein, 9 aa, synthetic construct
GGAGHDIAA

SEQ ID NO: 30875 - protein, 9 aa, synthetic construct
GGAGHDLAL

SEQ ID NO: 30876 - protein, 9 aa, synthetic construct
GGAGHDLIN

SEQ ID NO: 30877 - protein, 9 aa, synthetic construct
GGAGHDSIG

SEQ ID NO: 30878 - protein, 9 aa, synthetic construct
GGAGHDQIG

SEQ ID NO: 30879 - protein, 9 aa, synthetic construct
GGAGHDQIW

SEQ ID NO: 30880 - protein, 9 aa, synthetic construct
GGAGHDQIY

SEQ ID NO: 30881 - protein, 9 aa, synthetic construct
GGAGHDQLH

SEQ ID NO: 30882 - protein, 9 aa, synthetic construct
GGAGHDQLL

SEQ ID NO: 30883 - protein, 9 aa, synthetic construct
GGAGHDQLV

SEQ ID NO: 30884 - protein, 9 aa, synthetic construct
GGAGHDQVD

SEQ ID NO: 30885 - protein, 9 aa, synthetic construct
GGAGHDRFV

SEQ ID NO: 30886 - protein, 9 aa, synthetic construct
GGAGHDRII

SEQ ID NO: 30887 - protein, 9 aa, synthetic construct
GGAGHDRIN

SEQ ID NO: 30888 - protein, 9 aa, synthetic construct
GGAGHDRIV

SEQ ID NO: 30889 - protein, 9 aa, synthetic construct
GGAGHDRIW

SEQ ID NO: 30890 - protein, 9 aa, synthetic construct
GGAGHDRLR

SEQ ID NO: 30891 - protein, 9 aa, synthetic construct
GGAGHDRVH

SEQ ID NO: 30892 - protein, 9 aa, synthetic construct
GGAGHDSAD

SEQ ID NO: 30893 - protein, 9 aa, synthetic construct
GGAGHDSFG

SEQ ID NO: 30894 - protein, 9 aa, synthetic construct
GGAGHDSFI

SEQ ID NO: 30895 - protein, 9 aa, synthetic construct
GGAGHDSIE

SEQ ID NO: 30896 - protein, 9 aa, synthetic construct
GGAGHDQIS

SEQ ID NO: 30897 - protein, 9 aa, synthetic construct
GGAGHDNVV

SEQ ID NO: 30898 - protein, 9 aa, synthetic construct
GGAGHDLIS

SEQ ID NO: 30899 - protein, 9 aa, synthetic construct
GGAGHDNLY

SEQ ID NO: 30900 - protein, 9 aa, synthetic construct
GGAGHDLLG

SEQ ID NO: 30901 - protein, 9 aa, synthetic construct
GGAGHDLLW

SEQ ID NO: 30902 - protein, 9 aa, synthetic construct
GGAGHDLME

SEQ ID NO: 30903 - protein, 9 aa, synthetic construct
GGAGHDLVM

SEQ ID NO: 30904 - protein, 9 aa, synthetic construct
GGAGHDLVQ

SEQ ID NO: 30905 - protein, 9 aa, synthetic construct
GGAGHDLYQ

SEQ ID NO: 30906 - protein, 9 aa, synthetic construct
GGAGHDLYV

SEQ ID NO: 30907 - protein, 9 aa, synthetic construct
GGAGHDMAR

SEQ ID NO: 30908 - protein, 9 aa, synthetic construct
GGAGHDMAV

SEQ ID NO: 30909 - protein, 9 aa, synthetic construct
GGAGHDMID

SEQ ID NO: 30910 - protein, 9 aa, synthetic construct
GGAGHDMIM

SEQ ID NO: 30911 - protein, 9 aa, synthetic construct
GGAGHDMIS

SEQ ID NO: 30912 - protein, 9 aa, synthetic construct
GGAGHDMMD

SEQ ID NO: 30913 - protein, 9 aa, synthetic construct
GGAGHDNIS

SEQ ID NO: 30914 - protein, 9 aa, synthetic construct
GGAGHDNLG

SEQ ID NO: 30915 - protein, 9 aa, synthetic construct
GGAGHDNLN

SEQ ID NO: 30916 - protein, 9 aa, synthetic construct
GGAGHDNLQ

SEQ ID NO: 30917 - protein, 9 aa, synthetic construct
GGAGIDIIY

SEQ ID NO: 30918 - protein, 9 aa, synthetic construct
GGAGIDILE

SEQ ID NO: 30919 - protein, 9 aa, synthetic construct
GGAGEDVAY

SEQ ID NO: 30920 - protein, 9 aa, synthetic construct
GGAGIDWLR

SEQ ID NO: 30921 - protein, 9 aa, synthetic construct
GGAGIDVVR

SEQ ID NO: 30922 - protein, 9 aa, synthetic construct
GGAGIDVYI

SEQ ID NO: 30923 - protein, 9 aa, synthetic construct
GGAGIDWAS

SEQ ID NO: 30924 - protein, 9 aa, synthetic construct
GGAGIDWAT

SEQ ID NO: 30925 - protein, 9 aa, synthetic construct
GGAGIDWAY

SEQ ID NO: 30926 - protein, 9 aa, synthetic construct
GGAGIDWIS

SEQ ID NO: 30927 - protein, 9 aa, synthetic construct
GGAGIDWLA

SEQ ID NO: 30928 - protein, 9 aa, synthetic construct
GGAGIDWLF

SEQ ID NO: 30929 - protein, 9 aa, synthetic construct
GGAGIDYAG

SEQ ID NO: 30930 - protein, 9 aa, synthetic construct
GGAGIDILI

SEQ ID NO: 30931 - protein, 9 aa, synthetic construct
GGAGIDYAV

SEQ ID NO: 30932 - protein, 9 aa, synthetic construct
GGAGIDYIA

SEQ ID NO: 30933 - protein, 9 aa, synthetic construct
GGAGIDYLE

SEQ ID NO: 30934 - protein, 9 aa, synthetic construct
GGAGIDYLN

SEQ ID NO: 30935 - protein, 9 aa, synthetic construct
GGAGIDYLS

SEQ ID NO: 30936 - protein, 9 aa, synthetic construct
GGAGIDYVS

SEQ ID NO: 30937 - protein, 9 aa, synthetic construct
GGAGIDYVT

SEQ ID NO: 30938 - protein, 9 aa, synthetic construct
GGAGKDAAS

SEQ ID NO: 30939 - protein, 9 aa, synthetic construct
GGAGIDVMQ

SEQ ID NO: 30940 - protein, 9 aa, synthetic construct
GGAGIDVMN

SEQ ID NO: 30941 - protein, 9 aa, synthetic construct
GGAGIDVMF

SEQ ID NO: 30942 - protein, 9 aa, synthetic construct
GGAGIDVMA

SEQ ID NO: 30943 - protein, 9 aa, synthetic construct
GGAGIDTIT

SEQ ID NO: 30944 - protein, 9 aa, synthetic construct
GGAGIDTLM

SEQ ID NO: 30945 - protein, 9 aa, synthetic construct
GGAGIDTMQ

SEQ ID NO: 30946 - protein, 9 aa, synthetic construct
GGAGIDTMR

SEQ ID NO: 30947 - protein, 9 aa, synthetic construct
GGAGIDTVI

SEQ ID NO: 30948 - protein, 9 aa, synthetic construct
GGAGIDTVL

SEQ ID NO: 30949 - protein, 9 aa, synthetic construct
GGAGIDTVN

SEQ ID NO: 30950 - protein, 9 aa, synthetic construct
GGAGIDTVY

SEQ ID NO: 30951 - protein, 9 aa, synthetic construct
GGAGIDTYD

SEQ ID NO: 30952 - protein, 9 aa, synthetic construct
GGAGIDVAV

SEQ ID NO: 30953 - protein, 9 aa, synthetic construct
GGAGIDVFR

SEQ ID NO: 30954 - protein, 9 aa, synthetic construct
GGAGIDVIL

SEQ ID NO: 30955 - protein, 9 aa, synthetic construct
GGAGIDVIY

SEQ ID NO: 30956 - protein, 9 aa, synthetic construct
GGAGIDVLC

SEQ ID NO: 30957 - protein, 9 aa, synthetic construct
GGAGIDVLR

SEQ ID NO: 30958 - protein, 9 aa, synthetic construct
GGAGIDVLS

SEQ ID NO: 30959 - protein, 9 aa, synthetic construct
GGAGIDVLT

SEQ ID NO: 30960 - protein, 9 aa, synthetic construct
GGAGKDAFL

SEQ ID NO: 30961 - protein, 9 aa, synthetic construct
GGAGKDAFR

SEQ ID NO: 30962 - protein, 9 aa, synthetic construct
GGAGKDAIN

SEQ ID NO: 30963 - protein, 9 aa, synthetic construct
GGAGKDFAW

SEQ ID NO: 30964 - protein, 9 aa, synthetic construct
GGAGKDFFI

SEQ ID NO: 30965 - protein, 9 aa, synthetic construct
GGAGKDFFL

SEQ ID NO: 30966 - protein, 9 aa, synthetic construct
GGAGKDFIA

SEQ ID NO: 30967 - protein, 9 aa, synthetic construct
GGAGKDFIK

SEQ ID NO: 30968 - protein, 9 aa, synthetic construct
GGAGKDFLA

SEQ ID NO: 30969 - protein, 9 aa, synthetic construct
GGAGKDFLF

SEQ ID NO: 30970 - protein, 9 aa, synthetic construct
GGAGKDFVV

SEQ ID NO: 30971 - protein, 9 aa, synthetic construct
GGAGKDGAY

SEQ ID NO: 30972 - protein, 9 aa, synthetic construct
GGAGKDGFV

SEQ ID NO: 30973 - protein, 9 aa, synthetic construct
GGAGKDGIV

SEQ ID NO: 30974 - protein, 9 aa, synthetic construct
GGAGKDGLE

SEQ ID NO: 30975 - protein, 9 aa, synthetic construct
GGAGKDGMD

SEQ ID NO: 30976 - protein, 9 aa, synthetic construct
GGAGKDHFI

SEQ ID NO: 30977 - protein, 9 aa, synthetic construct
GGAGKDHLF

SEQ ID NO: 30978 - protein, 9 aa, synthetic construct
GGAGKDIFD

SEQ ID NO: 30979 - protein, 9 aa, synthetic construct
GGAGKDIFL

SEQ ID NO: 30980 - protein, 9 aa, synthetic construct
GGAGKDIMD

SEQ ID NO: 30981 - protein, 9 aa, synthetic construct
GGAGKDFAY

SEQ ID NO: 30982 - protein, 9 aa, synthetic construct
GGAGKDELT

SEQ ID NO: 30983 - protein, 9 aa, synthetic construct
GGAGKDAIS

SEQ ID NO: 30984 - protein, 9 aa, synthetic construct
GGAGKDELS

SEQ ID NO: 30985 - protein, 9 aa, synthetic construct
GGAGKDALD

SEQ ID NO: 30986 - protein, 9 aa, synthetic construct
GGAGKDALE

SEQ ID NO: 30987 - protein, 9 aa, synthetic construct
GGAGKDALF

SEQ ID NO: 30988 - protein, 9 aa, synthetic construct
GGAGKDALI

SEQ ID NO: 30989 - protein, 9 aa, synthetic construct
GGAGKDALL

SEQ ID NO: 30990 - protein, 9 aa, synthetic construct
GGAGKDALN

SEQ ID NO: 30991 - protein, 9 aa, synthetic construct
GGAGKDALQ

SEQ ID NO: 30992 - protein, 9 aa, synthetic construct
GGAGKDALS

SEQ ID NO: 30993 - protein, 9 aa, synthetic construct
GGAGKDAMR

SEQ ID NO: 30994 - protein, 9 aa, synthetic construct
GGAGKDAVN

SEQ ID NO: 30995 - protein, 9 aa, synthetic construct
GGAGKDDIK

SEQ ID NO: 30996 - protein, 9 aa, synthetic construct
GGAGKDDLS

SEQ ID NO: 30997 - protein, 9 aa, synthetic construct
GGAGKDDLT

SEQ ID NO: 30998 - protein, 9 aa, synthetic construct
GGAGKDDMV

SEQ ID NO: 30999 - protein, 9 aa, synthetic construct
GGAGKDEII

SEQ ID NO: 31000 - protein, 9 aa, synthetic construct
GGAGKDEIY

SEQ ID NO: 31001 - protein, 9 aa, synthetic construct
GGAGKDELQ

SEQ ID NO: 31002 - protein, 9 aa, synthetic construct
GGAGIDTIF

SEQ ID NO: 31003 - protein, 9 aa, synthetic construct
GGAGIDTIA

SEQ ID NO: 31004 - protein, 9 aa, synthetic construct
GGAGIDTFT

SEQ ID NO: 31005 - protein, 9 aa, synthetic construct
GGAGIDLMN

SEQ ID NO: 31006 - protein, 9 aa, synthetic construct
GGAGIDLMY

SEQ ID NO: 31007 - protein, 9 aa, synthetic construct
GGAGIDLVF

SEQ ID NO: 31008 - protein, 9 aa, synthetic construct
GGAGIDLVQ

SEQ ID NO: 31009 - protein, 9 aa, synthetic construct
GGAGIDLVS

SEQ ID NO: 31010 - protein, 9 aa, synthetic construct
GGAGIDMID

SEQ ID NO: 31011 - protein, 9 aa, synthetic construct
GGAGIDMLA

SEQ ID NO: 31012 - protein, 9 aa, synthetic construct
GGAGIDMLY

SEQ ID NO: 31013 - protein, 9 aa, synthetic construct
GGAGIDMMQ

SEQ ID NO: 31014 - protein, 9 aa, synthetic construct
GGAGIDMVD

SEQ ID NO: 31015 - protein, 9 aa, synthetic construct
GGAGIDNFK

SEQ ID NO: 31016 - protein, 9 aa, synthetic construct
GGAGIDNIA

SEQ ID NO: 31017 - protein, 9 aa, synthetic construct
GGAGIDNID

SEQ ID NO: 31018 - protein, 9 aa, synthetic construct
GGAGIDNLF

SEQ ID NO: 31019 - protein, 9 aa, synthetic construct
GGAGIDNLH

SEQ ID NO: 31020 - protein, 9 aa, synthetic construct
GGAGIDNLT

SEQ ID NO: 31021 - protein, 9 aa, synthetic construct
GGAGIDNMF

SEQ ID NO: 31022 - protein, 9 aa, synthetic construct
GGAGIDNMI

SEQ ID NO: 31023 - protein, 9 aa, synthetic construct
GGAGIDLMR

SEQ ID NO: 31024 - protein, 9 aa, synthetic construct
GGAGIDLMI

SEQ ID NO: 31025 - protein, 9 aa, synthetic construct
GGAGIDQAV

SEQ ID NO: 31026 - protein, 9 aa, synthetic construct
GGAGIDLMF

SEQ ID NO: 31027 - protein, 9 aa, synthetic construct
GGAGIDILK

SEQ ID NO: 31028 - protein, 9 aa, synthetic construct
GGAGIDILT

SEQ ID NO: 31029 - protein, 9 aa, synthetic construct
GGAGIDILY

SEQ ID NO: 31030 - protein, 9 aa, synthetic construct
GGAGIDIML

SEQ ID NO: 31031 - protein, 9 aa, synthetic construct
GGAGIDKLF

SEQ ID NO: 31032 - protein, 9 aa, synthetic construct
GGAGIDKLW

SEQ ID NO: 31033 - protein, 9 aa, synthetic construct
GGAGIDKLY

SEQ ID NO: 31034 - protein, 9 aa, synthetic construct
GGAGIDKVA

SEQ ID NO: 31035 - protein, 9 aa, synthetic construct
GGAGIDKVT

SEQ ID NO: 31036 - protein, 9 aa, synthetic construct
GGAGIDKVV

SEQ ID NO: 31037 - protein, 9 aa, synthetic construct
GGAGIDKVY

SEQ ID NO: 31038 - protein, 9 aa, synthetic construct
GGAGIDLAT

SEQ ID NO: 31039 - protein, 9 aa, synthetic construct
GGAGIDLID

SEQ ID NO: 31040 - protein, 9 aa, synthetic construct
GGAGIDLIE

SEQ ID NO: 31041 - protein, 9 aa, synthetic construct
GGAGIDLIL

SEQ ID NO: 31042 - protein, 9 aa, synthetic construct
GGAGIDLIN

SEQ ID NO: 31043 - protein, 9 aa, synthetic construct
GGAGIDLLS

SEQ ID NO: 31044 - protein, 9 aa, synthetic construct
GGAGIDNMT

SEQ ID NO: 31045 - protein, 9 aa, synthetic construct
GGAGIDQFQ

SEQ ID NO: 31046 - protein, 9 aa, synthetic construct
GGAGIDTFR

SEQ ID NO: 31047 - protein, 9 aa, synthetic construct
GGAGIDSFG

SEQ ID NO: 31048 - protein, 9 aa, synthetic construct
GGAGIDSIT

SEQ ID NO: 31049 - protein, 9 aa, synthetic construct
GGAGIDSLD

SEQ ID NO: 31050 - protein, 9 aa, synthetic construct
GGAGIDSLH

SEQ ID NO: 31051 - protein, 9 aa, synthetic construct
GGAGIDSLM

SEQ ID NO: 31052 - protein, 9 aa, synthetic construct
GGAGIDSLN

SEQ ID NO: 31053 - protein, 9 aa, synthetic construct
GGAGIDSLT

SEQ ID NO: 31054 - protein, 9 aa, synthetic construct
GGAGIDSMF

SEQ ID NO: 31055 - protein, 9 aa, synthetic construct
GGAGIDSMN

SEQ ID NO: 31056 - protein, 9 aa, synthetic construct
GGAGIDSMT

SEQ ID NO: 31057 - protein, 9 aa, synthetic construct
GGAGIDSYL

SEQ ID NO: 31058 - protein, 9 aa, synthetic construct
GGAGIDTAA

SEQ ID NO: 31059 - protein, 9 aa, synthetic construct
GGAGIDTAG

SEQ ID NO: 31060 - protein, 9 aa, synthetic construct
GGAGIDTAQ

SEQ ID NO: 31061 - protein, 9 aa, synthetic construct
GGAGIDTAR

SEQ ID NO: 31062 - protein, 9 aa, synthetic construct
GGAGIDTAT

SEQ ID NO: 31063 - protein, 9 aa, synthetic construct
GGAGIDTFA

SEQ ID NO: 31064 - protein, 9 aa, synthetic construct
GGAGIDTFD

SEQ ID NO: 31065 - protein, 9 aa, synthetic construct
GGAGIDSIK

SEQ ID NO: 31066 - protein, 9 aa, synthetic construct
GGAGIDSFA

SEQ ID NO: 31067 - protein, 9 aa, synthetic construct
GGAGIDQFV

SEQ ID NO: 31068 - protein, 9 aa, synthetic construct
GGAGIDSAS

SEQ ID NO: 31069 - protein, 9 aa, synthetic construct
GGAGIDQIA

SEQ ID NO: 31070 - protein, 9 aa, synthetic construct
GGAGIDQIS

SEQ ID NO: 31071 - protein, 9 aa, synthetic construct
GGAGIDQIT

SEQ ID NO: 31072 - protein, 9 aa, synthetic construct
GGAGIDQLI

SEQ ID NO: 31073 - protein, 9 aa, synthetic construct
GGAGIDQMA

SEQ ID NO: 31074 - protein, 9 aa, synthetic construct
GGAGIDQML

SEQ ID NO: 31075 - protein, 9 aa, synthetic construct
GGAGIDRAE

SEQ ID NO: 31076 - protein, 9 aa, synthetic construct
GGAGIDRAQ

SEQ ID NO: 31077 - protein, 9 aa, synthetic construct
GGAGIDRAY

SEQ ID NO: 31078 - protein, 9 aa, synthetic construct
GGAGIDRFF

SEQ ID NO: 31079 - protein, 9 aa, synthetic construct
GGAGIDRIN

SEQ ID NO: 31080 - protein, 9 aa, synthetic construct
GGAGIDRIW

SEQ ID NO: 31081 - protein, 9 aa, synthetic construct
GGAGIDRLS

SEQ ID NO: 31082 - protein, 9 aa, synthetic construct
GGAGIDRMD

SEQ ID NO: 31083 - protein, 9 aa, synthetic construct
GGAGIDRMF

SEQ ID NO: 31084 - protein, 9 aa, synthetic construct
GGAGIDRMW

SEQ ID NO: 31085 - protein, 9 aa, synthetic construct
GGAGIDRVI

SEQ ID NO: 31086 - protein, 9 aa, synthetic construct
GGAGHDFAC

SEQ ID NO: 31087 - protein, 9 aa, synthetic construct
GGAGHDELV

SEQ ID NO: 31088 - protein, 9 aa, synthetic construct
GGAGHDELT

SEQ ID NO: 31089 - protein, 9 aa, synthetic construct
GGAGFDTFD

SEQ ID NO: 31090 - protein, 9 aa, synthetic construct
GGAGFDSLW

SEQ ID NO: 31091 - protein, 9 aa, synthetic construct
GGAGFDSMS

SEQ ID NO: 31092 - protein, 9 aa, synthetic construct
GGAGFDSVI

SEQ ID NO: 31093 - protein, 9 aa, synthetic construct
GGAGFDTAA

SEQ ID NO: 31094 - protein, 9 aa, synthetic construct
GGAGFDTAG

SEQ ID NO: 31095 - protein, 9 aa, synthetic construct
GGAGFDTAH

SEQ ID NO: 31096 - protein, 9 aa, synthetic construct
GGAGFDTAI

SEQ ID NO: 31097 - protein, 9 aa, synthetic construct
GGAGFDTAR

SEQ ID NO: 31098 - protein, 9 aa, synthetic construct
GGAGFDTFR

SEQ ID NO: 31099 - protein, 9 aa, synthetic construct
GGAGHDELF

SEQ ID NO: 31100 - protein, 9 aa, synthetic construct
GGAGFDTIA

SEQ ID NO: 31101 - protein, 9 aa, synthetic construct
GGAGFDTIR

SEQ ID NO: 31102 - protein, 9 aa, synthetic construct
GGAGFDTLK

SEQ ID NO: 31103 - protein, 9 aa, synthetic construct
GGAGFDTLM

SEQ ID NO: 31104 - protein, 9 aa, synthetic construct
GGAGFDTLQ

SEQ ID NO: 31105 - protein, 9 aa, synthetic construct
GGAGFDTMM

SEQ ID NO: 31106 - protein, 9 aa, synthetic construct
GGAGFDTMN

SEQ ID NO: 31107 - protein, 9 aa, synthetic construct
GGAGFDTMR

SEQ ID NO: 31108 - protein, 9 aa, synthetic construct
GGAGFDSLT

SEQ ID NO: 31109 - protein, 9 aa, synthetic construct
GGAGFDSLS

SEQ ID NO: 31110 - protein, 9 aa, synthetic construct
GGAGFDSLE

SEQ ID NO: 31111 - protein, 9 aa, synthetic construct
GGAGFDSIV

SEQ ID NO: 31112 - protein, 9 aa, synthetic construct
GGAGFDQLS

SEQ ID NO: 31113 - protein, 9 aa, synthetic construct
GGAGFDQMT

SEQ ID NO: 31114 - protein, 9 aa, synthetic construct
GGAGFDQVY

SEQ ID NO: 31115 - protein, 9 aa, synthetic construct
GGAGFDRAD

SEQ ID NO: 31116 - protein, 9 aa, synthetic construct
GGAGFDRFF

SEQ ID NO: 31117 - protein, 9 aa, synthetic construct
GGAGFDRII

SEQ ID NO: 31118 - protein, 9 aa, synthetic construct
GGAGFDRIV

SEQ ID NO: 31119 - protein, 9 aa, synthetic construct
GGAGFDRIY

SEQ ID NO: 31120 - protein, 9 aa, synthetic construct
GGAGFDRLL

SEQ ID NO: 31121 - protein, 9 aa, synthetic construct
GGAGFDRLM

SEQ ID NO: 31122 - protein, 9 aa, synthetic construct
GGAGFDRLS

SEQ ID NO: 31123 - protein, 9 aa, synthetic construct
GGAGFDRMS

SEQ ID NO: 31124 - protein, 9 aa, synthetic construct
GGAGFDSFI

SEQ ID NO: 31125 - protein, 9 aa, synthetic construct
GGAGFDSFV

SEQ ID NO: 31126 - protein, 9 aa, synthetic construct
GGAGFDSID

SEQ ID NO: 31127 - protein, 9 aa, synthetic construct
GGAGFDSIF

SEQ ID NO: 31128 - protein, 9 aa, synthetic construct
GGAGFDSIL

SEQ ID NO: 31129 - protein, 9 aa, synthetic construct
GGAGFDTVH

SEQ ID NO: 31130 - protein, 9 aa, synthetic construct
GGAGFDTVL

SEQ ID NO: 31131 - protein, 9 aa, synthetic construct
GGAGFDTVN

SEQ ID NO: 31132 - protein, 9 aa, synthetic construct
GGAGGDAIS

SEQ ID NO: 31133 - protein, 9 aa, synthetic construct
GGAGGDALE

SEQ ID NO: 31134 - protein, 9 aa, synthetic construct
GGAGGDALH

SEQ ID NO: 31135 - protein, 9 aa, synthetic construct
GGAGGDALI

SEQ ID NO: 31136 - protein, 9 aa, synthetic construct
GGAGGDALL

SEQ ID NO: 31137 - protein, 9 aa, synthetic construct
GGAGGDALW

SEQ ID NO: 31138 - protein, 9 aa, synthetic construct
GGAGGDAMA

SEQ ID NO: 31139 - protein, 9 aa, synthetic construct
GGAGGDAMI

SEQ ID NO: 31140 - protein, 9 aa, synthetic construct
GGAGGDAMQ

SEQ ID NO: 31141 - protein, 9 aa, synthetic construct
GGAGGDAYV

SEQ ID NO: 31142 - protein, 9 aa, synthetic construct
GGAGGDCLY

SEQ ID NO: 31143 - protein, 9 aa, synthetic construct
GGAGGDDIE

SEQ ID NO: 31144 - protein, 9 aa, synthetic construct
GGAGGDDLQ

SEQ ID NO: 31145 - protein, 9 aa, synthetic construct
GGAGGDEFD

SEQ ID NO: 31146 - protein, 9 aa, synthetic construct
GGAGGDEFQ

SEQ ID NO: 31147 - protein, 9 aa, synthetic construct
GGAGGDEFV

SEQ ID NO: 31148 - protein, 9 aa, synthetic construct
GGAGGDEIH

SEQ ID NO: 31149 - protein, 9 aa, synthetic construct
GGAGGDEIL

SEQ ID NO: 31150 - protein, 9 aa, synthetic construct
GGAGGDALA

SEQ ID NO: 31151 - protein, 9 aa, synthetic construct
GGAGFDYLY

SEQ ID NO: 31152 - protein, 9 aa, synthetic construct
GGAGFDTYI

SEQ ID NO: 31153 - protein, 9 aa, synthetic construct
GGAGFDYLS

SEQ ID NO: 31154 - protein, 9 aa, synthetic construct
GGAGFDVAH

SEQ ID NO: 31155 - protein, 9 aa, synthetic construct
GGAGFDVAI

SEQ ID NO: 31156 - protein, 9 aa, synthetic construct
GGAGFDVFI

SEQ ID NO: 31157 - protein, 9 aa, synthetic construct
GGAGFDVFL

SEQ ID NO: 31158 - protein, 9 aa, synthetic construct
GGAGFDVFY

SEQ ID NO: 31159 - protein, 9 aa, synthetic construct
GGAGFDVIA

SEQ ID NO: 31160 - protein, 9 aa, synthetic construct
GGAGFDVLV

SEQ ID NO: 31161 - protein, 9 aa, synthetic construct
GGAGFDVLW

SEQ ID NO: 31162 - protein, 9 aa, synthetic construct
GGAGFDVLY

SEQ ID NO: 31163 - protein, 9 aa, synthetic construct
GGAGFDVVQ

SEQ ID NO: 31164 - protein, 9 aa, synthetic construct
GGAGFDVVR

SEQ ID NO: 31165 - protein, 9 aa, synthetic construct
GGAGFDWII

SEQ ID NO: 31166 - protein, 9 aa, synthetic construct
GGAGFDWLF

SEQ ID NO: 31167 - protein, 9 aa, synthetic construct
GGAGFDWMT

SEQ ID NO: 31168 - protein, 9 aa, synthetic construct
GGAGFDYAD

SEQ ID NO: 31169 - protein, 9 aa, synthetic construct
GGAGFDYAR

SEQ ID NO: 31170 - protein, 9 aa, synthetic construct
GGAGFDYLG

SEQ ID NO: 31171 - protein, 9 aa, synthetic construct
GGAGFDQID

SEQ ID NO: 31172 - protein, 9 aa, synthetic construct
GGAGFDQAS

SEQ ID NO: 31173 - protein, 9 aa, synthetic construct
GGAGFDNLR

SEQ ID NO: 31174 - protein, 9 aa, synthetic construct
GGAGEDYIE

SEQ ID NO: 31175 - protein, 9 aa, synthetic construct
GGAGEDYLA

SEQ ID NO: 31176 - protein, 9 aa, synthetic construct
GGAGEDYLK

SEQ ID NO: 31177 - protein, 9 aa, synthetic construct
GGAGEDYLN

SEQ ID NO: 31178 - protein, 9 aa, synthetic construct
GGAGEDYVR

SEQ ID NO: 31179 - protein, 9 aa, synthetic construct
GGAGFDAAD

SEQ ID NO: 31180 - protein, 9 aa, synthetic construct
GGAGFDAAS

SEQ ID NO: 31181 - protein, 9 aa, synthetic construct
GGAGFDAIE

SEQ ID NO: 31182 - protein, 9 aa, synthetic construct
GGAGFDALF

SEQ ID NO: 31183 - protein, 9 aa, synthetic construct
GGAGFDALN

SEQ ID NO: 31184 - protein, 9 aa, synthetic construct
GGAGFDALQ

SEQ ID NO: 31185 - protein, 9 aa, synthetic construct
GGAGFDALY

SEQ ID NO: 31186 - protein, 9 aa, synthetic construct
GGAGFDAMF

SEQ ID NO: 31187 - protein, 9 aa, synthetic construct
GGAGFDAYN

SEQ ID NO: 31188 - protein, 9 aa, synthetic construct
GGAGFDDLN

SEQ ID NO: 31189 - protein, 9 aa, synthetic construct
GGAGFDDMY

SEQ ID NO: 31190 - protein, 9 aa, synthetic construct
GGAGFDELD

SEQ ID NO: 31191 - protein, 9 aa, synthetic construct
GGAGFDELH

SEQ ID NO: 31192 - protein, 9 aa, synthetic construct
GGAGEDYIN

SEQ ID NO: 31193 - protein, 9 aa, synthetic construct
GGAGEDWLM

SEQ ID NO: 31194 - protein, 9 aa, synthetic construct
GGAGFDFLD

SEQ ID NO: 31195 - protein, 9 aa, synthetic construct
GGAGEDWIG

SEQ ID NO: 31196 - protein, 9 aa, synthetic construct
GGAGEDVFI

SEQ ID NO: 31197 - protein, 9 aa, synthetic construct
GGAGEDVFT

SEQ ID NO: 31198 - protein, 9 aa, synthetic construct
GGAGEDVIE

SEQ ID NO: 31199 - protein, 9 aa, synthetic construct
GGAGEDVIL

SEQ ID NO: 31200 - protein, 9 aa, synthetic construct
GGAGEDVIN

SEQ ID NO: 31201 - protein, 9 aa, synthetic construct
GGAGEDVIS

SEQ ID NO: 31202 - protein, 9 aa, synthetic construct
GGAGEDVIT

SEQ ID NO: 31203 - protein, 9 aa, synthetic construct
GGAGEDVLK

SEQ ID NO: 31204 - protein, 9 aa, synthetic construct
GGAGEDVLM

SEQ ID NO: 31205 - protein, 9 aa, synthetic construct
GGAGEDVLS

SEQ ID NO: 31206 - protein, 9 aa, synthetic construct
GGAGEDVLY

SEQ ID NO: 31207 - protein, 9 aa, synthetic construct
GGAGEDVMN

SEQ ID NO: 31208 - protein, 9 aa, synthetic construct
GGAGEDVMV

SEQ ID NO: 31209 - protein, 9 aa, synthetic construct
GGAGEDVVA

SEQ ID NO: 31210 - protein, 9 aa, synthetic construct
GGAGEDVVS

SEQ ID NO: 31211 - protein, 9 aa, synthetic construct
GGAGEDWAT

SEQ ID NO: 31212 - protein, 9 aa, synthetic construct
GGAGEDWIA

SEQ ID NO: 31213 - protein, 9 aa, synthetic construct
GGAGFDFLA

SEQ ID NO: 31214 - protein, 9 aa, synthetic construct
GGAGFDFLF

SEQ ID NO: 31215 - protein, 9 aa, synthetic construct
GGAGFDNLQ

SEQ ID NO: 31216 - protein, 9 aa, synthetic construct
GGAGFDLAD

SEQ ID NO: 31217 - protein, 9 aa, synthetic construct
GGAGFDLIE

SEQ ID NO: 31218 - protein, 9 aa, synthetic construct
GGAGFDLIF

SEQ ID NO: 31219 - protein, 9 aa, synthetic construct
GGAGFDLIG

SEQ ID NO: 31220 - protein, 9 aa, synthetic construct
GGAGFDLLA

SEQ ID NO: 31221 - protein, 9 aa, synthetic construct
GGAGFDLLD

SEQ ID NO: 31222 - protein, 9 aa, synthetic construct
GGAGFDLLK

SEQ ID NO: 31223 - protein, 9 aa, synthetic construct
GGAGFDLLN

SEQ ID NO: 31224 - protein, 9 aa, synthetic construct
GGAGFDLLR

SEQ ID NO: 31225 - protein, 9 aa, synthetic construct
GGAGFDLLV

SEQ ID NO: 31226 - protein, 9 aa, synthetic construct
GGAGFDLML

SEQ ID NO: 31227 - protein, 9 aa, synthetic construct
GGAGFDLVD

SEQ ID NO: 31228 - protein, 9 aa, synthetic construct
GGAGFDLVR

SEQ ID NO: 31229 - protein, 9 aa, synthetic construct
GGAGFDMAT

SEQ ID NO: 31230 - protein, 9 aa, synthetic construct
GGAGFDMIE

SEQ ID NO: 31231 - protein, 9 aa, synthetic construct
GGAGFDMLF

SEQ ID NO: 31232 - protein, 9 aa, synthetic construct
GGAGFDMVL

SEQ ID NO: 31233 - protein, 9 aa, synthetic construct
GGAGFDNAS

SEQ ID NO: 31234 - protein, 9 aa, synthetic construct
GGAGFDLAS

SEQ ID NO: 31235 - protein, 9 aa, synthetic construct
GGAGFDKMT

SEQ ID NO: 31236 - protein, 9 aa, synthetic construct
GGAGFDFVS

SEQ ID NO: 31237 - protein, 9 aa, synthetic construct
GGAGFDKLK

SEQ ID NO: 31238 - protein, 9 aa, synthetic construct
GGAGFDGVD

SEQ ID NO: 31239 - protein, 9 aa, synthetic construct
GGAGFDHLD

SEQ ID NO: 31240 - protein, 9 aa, synthetic construct
GGAGFDHLS

SEQ ID NO: 31241 - protein, 9 aa, synthetic construct
GGAGFDHLT

SEQ ID NO: 31242 - protein, 9 aa, synthetic construct
GGAGFDHLY

SEQ ID NO: 31243 - protein, 9 aa, synthetic construct
GGAGFDIAE

SEQ ID NO: 31244 - protein, 9 aa, synthetic construct
GGAGFDIAG

SEQ ID NO: 31245 - protein, 9 aa, synthetic construct
GGAGFDIAR

SEQ ID NO: 31246 - protein, 9 aa, synthetic construct
GGAGFDIAV

SEQ ID NO: 31247 - protein, 9 aa, synthetic construct
GGAGFDIAY

SEQ ID NO: 31248 - protein, 9 aa, synthetic construct
GGAGFDIFA

SEQ ID NO: 31249 - protein, 9 aa, synthetic construct
GGAGFDIID

SEQ ID NO: 31250 - protein, 9 aa, synthetic construct
GGAGFDIIE

SEQ ID NO: 31251 - protein, 9 aa, synthetic construct
GGAGFDIIF

SEQ ID NO: 31252 - protein, 9 aa, synthetic construct
GGAGFDILD

SEQ ID NO: 31253 - protein, 9 aa, synthetic construct
GGAGFDILF

SEQ ID NO: 31254 - protein, 9 aa, synthetic construct
GGAGFDIMT

SEQ ID NO: 31255 - protein, 9 aa, synthetic construct
GGAGGDEIY

SEQ ID NO: 31256 - protein, 9 aa, synthetic construct
GGAGGDELD

SEQ ID NO: 31257 - protein, 9 aa, synthetic construct
GGAGGDELE

SEQ ID NO: 31258 - protein, 9 aa, synthetic construct
GGAGGDTVF

SEQ ID NO: 31259 - protein, 9 aa, synthetic construct
GGAGGDTVV

SEQ ID NO: 31260 - protein, 9 aa, synthetic construct
GGAGGDTYH

SEQ ID NO: 31261 - protein, 9 aa, synthetic construct
GGAGGDTYI

SEQ ID NO: 31262 - protein, 9 aa, synthetic construct
GGAGGDTYL

SEQ ID NO: 31263 - protein, 9 aa, synthetic construct
GGAGGDTYY

SEQ ID NO: 31264 - protein, 9 aa, synthetic construct
GGAGGDVFD

SEQ ID NO: 31265 - protein, 9 aa, synthetic construct
GGAGGDVFE

SEQ ID NO: 31266 - protein, 9 aa, synthetic construct
GGAGGDVFL

SEQ ID NO: 31267 - protein, 9 aa, synthetic construct
GGAGGDVFM

SEQ ID NO: 31268 - protein, 9 aa, synthetic construct
GGAGGDVIA

SEQ ID NO: 31269 - protein, 9 aa, synthetic construct
GGAGGDVIT

SEQ ID NO: 31270 - protein, 9 aa, synthetic construct
GGAGGDVLK

SEQ ID NO: 31271 - protein, 9 aa, synthetic construct
GGAGGDVLL

SEQ ID NO: 31272 - protein, 9 aa, synthetic construct
GGAGGDVLQ

SEQ ID NO: 31273 - protein, 9 aa, synthetic construct
GGAGGDVMA

SEQ ID NO: 31274 - protein, 9 aa, synthetic construct
GGAGGDVMH

SEQ ID NO: 31275 - protein, 9 aa, synthetic construct
GGAGGDVMI

SEQ ID NO: 31276 - protein, 9 aa, synthetic construct
GGAGGDTVT

SEQ ID NO: 31277 - protein, 9 aa, synthetic construct
GGAGGDTMV

SEQ ID NO: 31278 - protein, 9 aa, synthetic construct
GGAGGDVMQ

SEQ ID NO: 31279 - protein, 9 aa, synthetic construct
GGAGGDTMN

SEQ ID NO: 31280 - protein, 9 aa, synthetic construct
GGAGGDSMQ

SEQ ID NO: 31281 - protein, 9 aa, synthetic construct
GGAGGDSMV

SEQ ID NO: 31282 - protein, 9 aa, synthetic construct
GGAGGDSVD

SEQ ID NO: 31283 - protein, 9 aa, synthetic construct
GGAGGDSVS

SEQ ID NO: 31284 - protein, 9 aa, synthetic construct
GGAGGDTFF

SEQ ID NO: 31285 - protein, 9 aa, synthetic construct
GGAGGDTFL

SEQ ID NO: 31286 - protein, 9 aa, synthetic construct
GGAGGDTFW

SEQ ID NO: 31287 - protein, 9 aa, synthetic construct
GGAGGDTIF

SEQ ID NO: 31288 - protein, 9 aa, synthetic construct
GGAGGDTII

SEQ ID NO: 31289 - protein, 9 aa, synthetic construct
GGAGGDTIK

SEQ ID NO: 31290 - protein, 9 aa, synthetic construct
GGAGGDTIL

SEQ ID NO: 31291 - protein, 9 aa, synthetic construct
GGAGGDTIN

SEQ ID NO: 31292 - protein, 9 aa, synthetic construct
GGAGGDTIV

SEQ ID NO: 31293 - protein, 9 aa, synthetic construct
GGAGGDTIY

SEQ ID NO: 31294 - protein, 9 aa, synthetic construct
GGAGGDTLW

SEQ ID NO: 31295 - protein, 9 aa, synthetic construct
GGAGGDTME

SEQ ID NO: 31296 - protein, 9 aa, synthetic construct
GGAGGDTMK

SEQ ID NO: 31297 - protein, 9 aa, synthetic construct
GGAGGDVML

SEQ ID NO: 31298 - protein, 9 aa, synthetic construct
GGAGGDVMR

SEQ ID NO: 31299 - protein, 9 aa, synthetic construct
GGAGGDSME

SEQ ID NO: 31300 - protein, 9 aa, synthetic construct
GGAGGDYVQ

SEQ ID NO: 31301 - protein, 9 aa, synthetic construct
GGAGHDAIS

SEQ ID NO: 31302 - protein, 9 aa, synthetic construct
GGAGHDAIY

SEQ ID NO: 31303 - protein, 9 aa, synthetic construct
GGAGHDALD

SEQ ID NO: 31304 - protein, 9 aa, synthetic construct
GGAGHDALG

SEQ ID NO: 31305 - protein, 9 aa, synthetic construct
GGAGHDALH

SEQ ID NO: 31306 - protein, 9 aa, synthetic construct
GGAGHDALQ

SEQ ID NO: 31307 - protein, 9 aa, synthetic construct
GGAGHDALS

SEQ ID NO: 31308 - protein, 9 aa, synthetic construct
GGAGHDAMI

SEQ ID NO: 31309 - protein, 9 aa, synthetic construct
GGAGHDAVK

SEQ ID NO: 31310 - protein, 9 aa, synthetic construct
GGAGHDDAT

SEQ ID NO: 31311 - protein, 9 aa, synthetic construct
GGAGHDDVQ

SEQ ID NO: 31312 - protein, 9 aa, synthetic construct
GGAGHDEAR

SEQ ID NO: 31313 - protein, 9 aa, synthetic construct
GGAGHDEAS

SEQ ID NO: 31314 - protein, 9 aa, synthetic construct
GGAGHDEFI

SEQ ID NO: 31315 - protein, 9 aa, synthetic construct
GGAGHDEIA

SEQ ID NO: 31316 - protein, 9 aa, synthetic construct
GGAGHDEIY

SEQ ID NO: 31317 - protein, 9 aa, synthetic construct
GGAGHDELA

SEQ ID NO: 31318 - protein, 9 aa, synthetic construct
GGAGHDAID

SEQ ID NO: 31319 - protein, 9 aa, synthetic construct
GGAGGDYMQ

SEQ ID NO: 31320 - protein, 9 aa, synthetic construct
GGAGGDWID

SEQ ID NO: 31321 - protein, 9 aa, synthetic construct
GGAGGDYLV

SEQ ID NO: 31322 - protein, 9 aa, synthetic construct
GGAGGDWIE

SEQ ID NO: 31323 - protein, 9 aa, synthetic construct
GGAGGDWIG

SEQ ID NO: 31324 - protein, 9 aa, synthetic construct
GGAGGDWIN

SEQ ID NO: 31325 - protein, 9 aa, synthetic construct
GGAGGDWIS

SEQ ID NO: 31326 - protein, 9 aa, synthetic construct
GGAGGDWLI

SEQ ID NO: 31327 - protein, 9 aa, synthetic construct
GGAGGDWLN

SEQ ID NO: 31328 - protein, 9 aa, synthetic construct
GGAGGDWLQ

SEQ ID NO: 31329 - protein, 9 aa, synthetic construct
GGAGGDWLY

SEQ ID NO: 31330 - protein, 9 aa, synthetic construct
GGAGGDWME

SEQ ID NO: 31331 - protein, 9 aa, synthetic construct
GGAGGDYAS

SEQ ID NO: 31332 - protein, 9 aa, synthetic construct
GGAGGDYFV

SEQ ID NO: 31333 - protein, 9 aa, synthetic construct
GGAGGDYIE

SEQ ID NO: 31334 - protein, 9 aa, synthetic construct
GGAGGDYIL

SEQ ID NO: 31335 - protein, 9 aa, synthetic construct
GGAGGDYLA

SEQ ID NO: 31336 - protein, 9 aa, synthetic construct
GGAGGDYLE

SEQ ID NO: 31337 - protein, 9 aa, synthetic construct
GGAGGDYLH

SEQ ID NO: 31338 - protein, 9 aa, synthetic construct
GGAGGDYLM

SEQ ID NO: 31339 - protein, 9 aa, synthetic construct
GGAGGDSMK

SEQ ID NO: 31340 - protein, 9 aa, synthetic construct
GGAGGDSLL

SEQ ID NO: 31341 - protein, 9 aa, synthetic construct
GGAGGDELF

SEQ ID NO: 31342 - protein, 9 aa, synthetic construct
GGAGGDHLL

SEQ ID NO: 31343 - protein, 9 aa, synthetic construct
GGAGGDHLS

SEQ ID NO: 31344 - protein, 9 aa, synthetic construct
GGAGGDHLY

SEQ ID NO: 31345 - protein, 9 aa, synthetic construct
GGAGGDIIA

SEQ ID NO: 31346 - protein, 9 aa, synthetic construct
GGAGGDIIK

SEQ ID NO: 31347 - protein, 9 aa, synthetic construct
GGAGGDILE

SEQ ID NO: 31348 - protein, 9 aa, synthetic construct
GGAGGDILG

SEQ ID NO: 31349 - protein, 9 aa, synthetic construct
GGAGGDILK

SEQ ID NO: 31350 - protein, 9 aa, synthetic construct
GGAGGDILR

SEQ ID NO: 31351 - protein, 9 aa, synthetic construct
GGAGGDIVA

SEQ ID NO: 31352 - protein, 9 aa, synthetic construct
GGAGGDIYI

SEQ ID NO: 31353 - protein, 9 aa, synthetic construct
GGAGGDKAL

SEQ ID NO: 31354 - protein, 9 aa, synthetic construct
GGAGGDKIF

SEQ ID NO: 31355 - protein, 9 aa, synthetic construct
GGAGGDKIN

SEQ ID NO: 31356 - protein, 9 aa, synthetic construct
GGAGGDKLL

SEQ ID NO: 31357 - protein, 9 aa, synthetic construct
GGAGGDKMF

SEQ ID NO: 31358 - protein, 9 aa, synthetic construct
GGAGGDLFL

SEQ ID NO: 31359 - protein, 9 aa, synthetic construct
GGAGGDLIK

SEQ ID NO: 31360 - protein, 9 aa, synthetic construct
GGAGGDHLN

SEQ ID NO: 31361 - protein, 9 aa, synthetic construct
GGAGGDHLF

SEQ ID NO: 31362 - protein, 9 aa, synthetic construct
GGAGGDLIY

SEQ ID NO: 31363 - protein, 9 aa, synthetic construct
GGAGGDHII

SEQ ID NO: 31364 - protein, 9 aa, synthetic construct
GGAGGDELG

SEQ ID NO: 31365 - protein, 9 aa, synthetic construct
GGAGGDELT

SEQ ID NO: 31366 - protein, 9 aa, synthetic construct
GGAGGDEMH

SEQ ID NO: 31367 - protein, 9 aa, synthetic construct
GGAGGDEMR

SEQ ID NO: 31368 - protein, 9 aa, synthetic construct
GGAGGDFAD

SEQ ID NO: 31369 - protein, 9 aa, synthetic construct
GGAGGDFAS

SEQ ID NO: 31370 - protein, 9 aa, synthetic construct
GGAGGDFLL

SEQ ID NO: 31371 - protein, 9 aa, synthetic construct
GGAGGDFLM

SEQ ID NO: 31372 - protein, 9 aa, synthetic construct
GGAGGDFLN

SEQ ID NO: 31373 - protein, 9 aa, synthetic construct
GGAGGDFLT

SEQ ID NO: 31374 - protein, 9 aa, synthetic construct
GGAGGDFMF

SEQ ID NO: 31375 - protein, 9 aa, synthetic construct
GGAGGDFVQ

SEQ ID NO: 31376 - protein, 9 aa, synthetic construct
GGAGGDFVV

SEQ ID NO: 31377 - protein, 9 aa, synthetic construct
GGAGGDGAD

SEQ ID NO: 31378 - protein, 9 aa, synthetic construct
GGAGGDGLF

SEQ ID NO: 31379 - protein, 9 aa, synthetic construct
GGAGGDGLT

SEQ ID NO: 31380 - protein, 9 aa, synthetic construct
GGAGGDHFI

SEQ ID NO: 31381 - protein, 9 aa, synthetic construct
GGAGGDLIV

SEQ ID NO: 31382 - protein, 9 aa, synthetic construct
GGAGGDLLM

SEQ ID NO: 31383 - protein, 9 aa, synthetic construct
GGAGGDSLK

SEQ ID NO: 31384 - protein, 9 aa, synthetic construct
GGAGGDQMV

SEQ ID NO: 31385 - protein, 9 aa, synthetic construct
GGAGGDRAS

SEQ ID NO: 31386 - protein, 9 aa, synthetic construct
GGAGGDRAY

SEQ ID NO: 31387 - protein, 9 aa, synthetic construct
GGAGGDRFD

SEQ ID NO: 31388 - protein, 9 aa, synthetic construct
GGAGGDRIA

SEQ ID NO: 31389 - protein, 9 aa, synthetic construct
GGAGGDRIS

SEQ ID NO: 31390 - protein, 9 aa, synthetic construct
GGAGGDRLW

SEQ ID NO: 31391 - protein, 9 aa, synthetic construct
GGAGGDRMA

SEQ ID NO: 31392 - protein, 9 aa, synthetic construct
GGAGGDRME

SEQ ID NO: 31393 - protein, 9 aa, synthetic construct
GGAGGDRMI

SEQ ID NO: 31394 - protein, 9 aa, synthetic construct
GGAGGDRML

SEQ ID NO: 31395 - protein, 9 aa, synthetic construct
GGAGGDRMM

SEQ ID NO: 31396 - protein, 9 aa, synthetic construct
GGAGGDRMT

SEQ ID NO: 31397 - protein, 9 aa, synthetic construct
GGAGGDRMY

SEQ ID NO: 31398 - protein, 9 aa, synthetic construct
GGAGGDRYY

SEQ ID NO: 31399 - protein, 9 aa, synthetic construct
GGAGGDSAD

SEQ ID NO: 31400 - protein, 9 aa, synthetic construct
GGAGGDSFV

SEQ ID NO: 31401 - protein, 9 aa, synthetic construct
GGAGGDSIL

SEQ ID NO: 31402 - protein, 9 aa, synthetic construct
GGAGGDQVI

SEQ ID NO: 31403 - protein, 9 aa, synthetic construct
GGAGGDQMF

SEQ ID NO: 31404 - protein, 9 aa, synthetic construct
GGAGGDLLR

SEQ ID NO: 31405 - protein, 9 aa, synthetic construct
GGAGGDQLK

SEQ ID NO: 31406 - protein, 9 aa, synthetic construct
GGAGGDLMA

SEQ ID NO: 31407 - protein, 9 aa, synthetic construct
GGAGGDLMF

SEQ ID NO: 31408 - protein, 9 aa, synthetic construct
GGAGGDLMK

SEQ ID NO: 31409 - protein, 9 aa, synthetic construct
GGAGGDMAV

SEQ ID NO: 31410 - protein, 9 aa, synthetic construct
GGAGGDMLS

SEQ ID NO: 31411 - protein, 9 aa, synthetic construct
GGAGGDMMR

SEQ ID NO: 31412 - protein, 9 aa, synthetic construct
GGAGGDNIT

SEQ ID NO: 31413 - protein, 9 aa, synthetic construct
GGAGGDNLD

SEQ ID NO: 31414 - protein, 9 aa, synthetic construct
GGAGGDNLH

SEQ ID NO: 31415 - protein, 9 aa, synthetic construct
GGAGGDNLR

SEQ ID NO: 31416 - protein, 9 aa, synthetic construct
GGAGGDNLS

SEQ ID NO: 31417 - protein, 9 aa, synthetic construct
GGAGGDNLV

SEQ ID NO: 31418 - protein, 9 aa, synthetic construct
GGAGGDNMD

SEQ ID NO: 31419 - protein, 9 aa, synthetic construct
GGAGGDQFI

SEQ ID NO: 31420 - protein, 9 aa, synthetic construct
GGAGGDQIK

SEQ ID NO: 31421 - protein, 9 aa, synthetic construct
GGAGGDQIW

SEQ ID NO: 31422 - protein, 9 aa, synthetic construct
GGAGGDQLE

SEQ ID NO: 31423 - protein, 9 aa, synthetic construct
GGAGTDRFT

SEQ ID NO: 31424 - protein, 9 aa, synthetic construct
GGAGTDRFV

SEQ ID NO: 31425 - protein, 9 aa, synthetic construct
GGAGTDRLR

SEQ ID NO: 31426 - protein, 9 aa, synthetic construct
GGDGNDRIQ

SEQ ID NO: 31427 - protein, 9 aa, synthetic construct
GGDGNDQMT

SEQ ID NO: 31428 - protein, 9 aa, synthetic construct
GGDGNDQVW

SEQ ID NO: 31429 - protein, 9 aa, synthetic construct
GGDGNDQYR

SEQ ID NO: 31430 - protein, 9 aa, synthetic construct
GGDGNDRFI

SEQ ID NO: 31431 - protein, 9 aa, synthetic construct
GGDGNDRFM

SEQ ID NO: 31432 - protein, 9 aa, synthetic construct
GGDGNDRFN

SEQ ID NO: 31433 - protein, 9 aa, synthetic construct
GGDGNDRFQ

SEQ ID NO: 31434 - protein, 9 aa, synthetic construct
GGDGNDRII

SEQ ID NO: 31435 - protein, 9 aa, synthetic construct
GGDGNDRIW

SEQ ID NO: 31436 - protein, 9 aa, synthetic construct
GGDGNDVFE

SEQ ID NO: 31437 - protein, 9 aa, synthetic construct
GGDGNDRLC

SEQ ID NO: 31438 - protein, 9 aa, synthetic construct
GGDGNDRMG

SEQ ID NO: 31439 - protein, 9 aa, synthetic construct
GGDGNDRMH

SEQ ID NO: 31440 - protein, 9 aa, synthetic construct
GGDGNDRML

SEQ ID NO: 31441 - protein, 9 aa, synthetic construct
GGDGNDRMN

SEQ ID NO: 31442 - protein, 9 aa, synthetic construct
GGDGNDRMR

SEQ ID NO: 31443 - protein, 9 aa, synthetic construct
GGDGNDRMW

SEQ ID NO: 31444 - protein, 9 aa, synthetic construct
GGDGNDRVA

SEQ ID NO: 31445 - protein, 9 aa, synthetic construct
GGDGNDQML

SEQ ID NO: 31446 - protein, 9 aa, synthetic construct
GGDGNDQMD

SEQ ID NO: 31447 - protein, 9 aa, synthetic construct
GGDGNDQLQ

SEQ ID NO: 31448 - protein, 9 aa, synthetic construct
GGDGNDQIT

SEQ ID NO: 31449 - protein, 9 aa, synthetic construct
GGDGNDNIV

SEQ ID NO: 31450 - protein, 9 aa, synthetic construct
GGDGNDNIW

SEQ ID NO: 31451 - protein, 9 aa, synthetic construct
GGDGNDNIY

SEQ ID NO: 31452 - protein, 9 aa, synthetic construct
GGDGNDNLE

SEQ ID NO: 31453 - protein, 9 aa, synthetic construct
GGDGNDNMG

SEQ ID NO: 31454 - protein, 9 aa, synthetic construct
GGDGNDNMR

SEQ ID NO: 31455 - protein, 9 aa, synthetic construct
GGDGNDNVA

SEQ ID NO: 31456 - protein, 9 aa, synthetic construct
GGDGNDNVD

SEQ ID NO: 31457 - protein, 9 aa, synthetic construct
GGDGNDNVF

SEQ ID NO: 31458 - protein, 9 aa, synthetic construct
GGDGNDNVQ

SEQ ID NO: 31459 - protein, 9 aa, synthetic construct
GGDGNDNYI

SEQ ID NO: 31460 - protein, 9 aa, synthetic construct
GGDGNDNYL

SEQ ID NO: 31461 - protein, 9 aa, synthetic construct
GGDGNDNYY

SEQ ID NO: 31462 - protein, 9 aa, synthetic construct
GGDGNDQAD

SEQ ID NO: 31463 - protein, 9 aa, synthetic construct
GGDGNDQFF

SEQ ID NO: 31464 - protein, 9 aa, synthetic construct
GGDGNDQIL

SEQ ID NO: 31465 - protein, 9 aa, synthetic construct
GGDGNDQIM

SEQ ID NO: 31466 - protein, 9 aa, synthetic construct
GGDGNDRVK

SEQ ID NO: 31467 - protein, 9 aa, synthetic construct
GGDGNDRYI

SEQ ID NO: 31468 - protein, 9 aa, synthetic construct
GGDGNDRYL

SEQ ID NO: 31469 - protein, 9 aa, synthetic construct
GGDGNDTAW

SEQ ID NO: 31470 - protein, 9 aa, synthetic construct
GGDGNDTFG

SEQ ID NO: 31471 - protein, 9 aa, synthetic construct
GGDGNDTFQ

SEQ ID NO: 31472 - protein, 9 aa, synthetic construct
GGDGNDTIC

SEQ ID NO: 31473 - protein, 9 aa, synthetic construct
GGDGNDTLC

SEQ ID NO: 31474 - protein, 9 aa, synthetic construct
GGDGNDTMM

SEQ ID NO: 31475 - protein, 9 aa, synthetic construct
GGDGNDTMQ

SEQ ID NO: 31476 - protein, 9 aa, synthetic construct
GGDGNDTMW

SEQ ID NO: 31477 - protein, 9 aa, synthetic construct
GGDGNDTVE

SEQ ID NO: 31478 - protein, 9 aa, synthetic construct
GGDGNDTVH

SEQ ID NO: 31479 - protein, 9 aa, synthetic construct
GGDGNDTVQ

SEQ ID NO: 31480 - protein, 9 aa, synthetic construct
GGDGNDTYA

SEQ ID NO: 31481 - protein, 9 aa, synthetic construct
GGDGNDTYK

SEQ ID NO: 31482 - protein, 9 aa, synthetic construct
GGDGNDTYQ

SEQ ID NO: 31483 - protein, 9 aa, synthetic construct
GGDGNDVAA

SEQ ID NO: 31484 - protein, 9 aa, synthetic construct
GGDGNDVAE

SEQ ID NO: 31485 - protein, 9 aa, synthetic construct
GGDGNDVAQ

SEQ ID NO: 31486 - protein, 9 aa, synthetic construct
GGDGNDVAV

SEQ ID NO: 31487 - protein, 9 aa, synthetic construct
GGDGNDTFD

SEQ ID NO: 31488 - protein, 9 aa, synthetic construct
GGDGNDTAG

SEQ ID NO: 31489 - protein, 9 aa, synthetic construct
GGDGNDSAF

SEQ ID NO: 31490 - protein, 9 aa, synthetic construct
GGDGNDSYL

SEQ ID NO: 31491 - protein, 9 aa, synthetic construct
GGDGNDSAK

SEQ ID NO: 31492 - protein, 9 aa, synthetic construct
GGDGNDSAR

SEQ ID NO: 31493 - protein, 9 aa, synthetic construct
GGDGNDSAS

SEQ ID NO: 31494 - protein, 9 aa, synthetic construct
GGDGNDSAW

SEQ ID NO: 31495 - protein, 9 aa, synthetic construct
GGDGNDSFD

SEQ ID NO: 31496 - protein, 9 aa, synthetic construct
GGDGNDSFL

SEQ ID NO: 31497 - protein, 9 aa, synthetic construct
GGDGNDSFN

SEQ ID NO: 31498 - protein, 9 aa, synthetic construct
GGDGNDSFS

SEQ ID NO: 31499 - protein, 9 aa, synthetic construct
GGDGNDSIK

SEQ ID NO: 31500 - protein, 9 aa, synthetic construct
GGDGNDSIR

SEQ ID NO: 31501 - protein, 9 aa, synthetic construct
GGDGNDSLK

SEQ ID NO: 31502 - protein, 9 aa, synthetic construct
GGDGNDSMD

SEQ ID NO: 31503 - protein, 9 aa, synthetic construct
GGDGNDSMF

SEQ ID NO: 31504 - protein, 9 aa, synthetic construct
GGDGNDSMM

SEQ ID NO: 31505 - protein, 9 aa, synthetic construct
GGDGNDSVG

SEQ ID NO: 31506 - protein, 9 aa, synthetic construct
GGDGNDSVQ

SEQ ID NO: 31507 - protein, 9 aa, synthetic construct
GGDGNDSVV

SEQ ID NO: 31508 - protein, 9 aa, synthetic construct
GGDGNDNIS

SEQ ID NO: 31509 - protein, 9 aa, synthetic construct
GGDGNDNIK

SEQ ID NO: 31510 - protein, 9 aa, synthetic construct
GGDGNDNII

SEQ ID NO: 31511 - protein, 9 aa, synthetic construct
GGDGNDHMI

SEQ ID NO: 31512 - protein, 9 aa, synthetic construct
GGDGNDHMV

SEQ ID NO: 31513 - protein, 9 aa, synthetic construct
GGDGNDHVH

SEQ ID NO: 31514 - protein, 9 aa, synthetic construct
GGDGNDHVV

SEQ ID NO: 31515 - protein, 9 aa, synthetic construct
GGDGNDIAA

SEQ ID NO: 31516 - protein, 9 aa, synthetic construct
GGDGNDIAE

SEQ ID NO: 31517 - protein, 9 aa, synthetic construct
GGDGNDIAN

SEQ ID NO: 31518 - protein, 9 aa, synthetic construct
GGDGNDIAY

SEQ ID NO: 31519 - protein, 9 aa, synthetic construct
GGDGNDIFI

SEQ ID NO: 31520 - protein, 9 aa, synthetic construct
GGDGNDIFQ

SEQ ID NO: 31521 - protein, 9 aa, synthetic construct
GGDGNDIFR

SEQ ID NO: 31522 - protein, 9 aa, synthetic construct
GGDGNDIFT

SEQ ID NO: 31523 - protein, 9 aa, synthetic construct
GGDGNDIFY

SEQ ID NO: 31524 - protein, 9 aa, synthetic construct
GGDGNDIIV

SEQ ID NO: 31525 - protein, 9 aa, synthetic construct
GGDGNDIMF

SEQ ID NO: 31526 - protein, 9 aa, synthetic construct
GGDGNDIMG

SEQ ID NO: 31527 - protein, 9 aa, synthetic construct
GGDGNDIMQ

SEQ ID NO: 31528 - protein, 9 aa, synthetic construct
GGDGNDIMS

SEQ ID NO: 31529 - protein, 9 aa, synthetic construct
GGDGNDHMT

SEQ ID NO: 31530 - protein, 9 aa, synthetic construct
GGDGNDHMF

SEQ ID NO: 31531 - protein, 9 aa, synthetic construct
GGDGNDIVK

SEQ ID NO: 31532 - protein, 9 aa, synthetic construct
GGDGNDHLQ

SEQ ID NO: 31533 - protein, 9 aa, synthetic construct
GGDGNDGII

SEQ ID NO: 31534 - protein, 9 aa, synthetic construct
GGDGNDGIQ

SEQ ID NO: 31535 - protein, 9 aa, synthetic construct
GGDGNDGIV

SEQ ID NO: 31536 - protein, 9 aa, synthetic construct
GGDGNDGIW

SEQ ID NO: 31537 - protein, 9 aa, synthetic construct
GGDGNDGLE

SEQ ID NO: 31538 - protein, 9 aa, synthetic construct
GGDGNDGLK

SEQ ID NO: 31539 - protein, 9 aa, synthetic construct
GGDGNDGLL

SEQ ID NO: 31540 - protein, 9 aa, synthetic construct
GGDGNDGLT

SEQ ID NO: 31541 - protein, 9 aa, synthetic construct
GGDGNDGLW

SEQ ID NO: 31542 - protein, 9 aa, synthetic construct
GGDGNDGMA

SEQ ID NO: 31543 - protein, 9 aa, synthetic construct
GGDGNDGMN

SEQ ID NO: 31544 - protein, 9 aa, synthetic construct
GGDGNDGMR

SEQ ID NO: 31545 - protein, 9 aa, synthetic construct
GGDGNDGMS

SEQ ID NO: 31546 - protein, 9 aa, synthetic construct
GGDGNDHAN

SEQ ID NO: 31547 - protein, 9 aa, synthetic construct
GGDGNDHIE

SEQ ID NO: 31548 - protein, 9 aa, synthetic construct
GGDGNDHIT

SEQ ID NO: 31549 - protein, 9 aa, synthetic construct
GGDGNDHLM

SEQ ID NO: 31550 - protein, 9 aa, synthetic construct
GGDGNDIVD

SEQ ID NO: 31551 - protein, 9 aa, synthetic construct
GGDGNDIVS

SEQ ID NO: 31552 - protein, 9 aa, synthetic construct
GGDGNDNIE

SEQ ID NO: 31553 - protein, 9 aa, synthetic construct
GGDGNDLMV

SEQ ID NO: 31554 - protein, 9 aa, synthetic construct
GGDGNDLVA

SEQ ID NO: 31555 - protein, 9 aa, synthetic construct
GGDGNDLVL

SEQ ID NO: 31556 - protein, 9 aa, synthetic construct
GGDGNDLVR

SEQ ID NO: 31557 - protein, 9 aa, synthetic construct
GGDGNDLVV

SEQ ID NO: 31558 - protein, 9 aa, synthetic construct
GGDGNDLYK

SEQ ID NO: 31559 - protein, 9 aa, synthetic construct
GGDGNDMAT

SEQ ID NO: 31560 - protein, 9 aa, synthetic construct
GGDGNDMIA

SEQ ID NO: 31561 - protein, 9 aa, synthetic construct
GGDGNDMII

SEQ ID NO: 31562 - protein, 9 aa, synthetic construct
GGDGNDMIS

SEQ ID NO: 31563 - protein, 9 aa, synthetic construct
GGDGNDMLA

SEQ ID NO: 31564 - protein, 9 aa, synthetic construct
GGDGNDMLK

SEQ ID NO: 31565 - protein, 9 aa, synthetic construct
GGDGNDMLV

SEQ ID NO: 31566 - protein, 9 aa, synthetic construct
GGDGNDMVA

SEQ ID NO: 31567 - protein, 9 aa, synthetic construct
GGDGNDMVY

SEQ ID NO: 31568 - protein, 9 aa, synthetic construct
GGDGNDMYF

SEQ ID NO: 31569 - protein, 9 aa, synthetic construct
GGDGNDNAY

SEQ ID NO: 31570 - protein, 9 aa, synthetic construct
GGDGNDNFT

SEQ ID NO: 31571 - protein, 9 aa, synthetic construct
GGDGNDLMW

SEQ ID NO: 31572 - protein, 9 aa, synthetic construct
GGDGNDLMQ

SEQ ID NO: 31573 - protein, 9 aa, synthetic construct
GGDGNDIYE

SEQ ID NO: 31574 - protein, 9 aa, synthetic construct
GGDGNDLMG

SEQ ID NO: 31575 - protein, 9 aa, synthetic construct
GGDGNDIYM

SEQ ID NO: 31576 - protein, 9 aa, synthetic construct
GGDGNDIYT

SEQ ID NO: 31577 - protein, 9 aa, synthetic construct
GGDGNDKFV

SEQ ID NO: 31578 - protein, 9 aa, synthetic construct
GGDGNDKIA

SEQ ID NO: 31579 - protein, 9 aa, synthetic construct
GGDGNDKIG

SEQ ID NO: 31580 - protein, 9 aa, synthetic construct
GGDGNDKIH

SEQ ID NO: 31581 - protein, 9 aa, synthetic construct
GGDGNDKII

SEQ ID NO: 31582 - protein, 9 aa, synthetic construct
GGDGNDKLH

SEQ ID NO: 31583 - protein, 9 aa, synthetic construct
GGDGNDKLW

SEQ ID NO: 31584 - protein, 9 aa, synthetic construct
GGDGNDKMF

SEQ ID NO: 31585 - protein, 9 aa, synthetic construct
GGDGNDKVR

SEQ ID NO: 31586 - protein, 9 aa, synthetic construct
GGDGNDKVV

SEQ ID NO: 31587 - protein, 9 aa, synthetic construct
GGDGNDKVY

SEQ ID NO: 31588 - protein, 9 aa, synthetic construct
GGDGNDLAF

SEQ ID NO: 31589 - protein, 9 aa, synthetic construct
GGDGNDLIK

SEQ ID NO: 31590 - protein, 9 aa, synthetic construct
GGDGNDLIM

SEQ ID NO: 31591 - protein, 9 aa, synthetic construct
GGDGNDLIW

SEQ ID NO: 31592 - protein, 9 aa, synthetic construct
GGDGNDVAY

SEQ ID NO: 31593 - protein, 9 aa, synthetic construct
GGDGNDVFF

SEQ ID NO: 31594 - protein, 9 aa, synthetic construct
GGDGRDDIY

SEQ ID NO: 31595 - protein, 9 aa, synthetic construct
GGDGQDRLI

SEQ ID NO: 31596 - protein, 9 aa, synthetic construct
GGDGQDQLF

SEQ ID NO: 31597 - protein, 9 aa, synthetic construct
GGDGQDQLS

SEQ ID NO: 31598 - protein, 9 aa, synthetic construct
GGDGQDQLY

SEQ ID NO: 31599 - protein, 9 aa, synthetic construct
GGDGQDRFF

SEQ ID NO: 31600 - protein, 9 aa, synthetic construct
GGDGQDRFV

SEQ ID NO: 31601 - protein, 9 aa, synthetic construct
GGDGQDRIL

SEQ ID NO: 31602 - protein, 9 aa, synthetic construct
GGDGQDRLD

SEQ ID NO: 31603 - protein, 9 aa, synthetic construct
GGDGQDRLE

SEQ ID NO: 31604 - protein, 9 aa, synthetic construct
GGDGQDRLQ

SEQ ID NO: 31605 - protein, 9 aa, synthetic construct
GGDGNDVFH

SEQ ID NO: 31606 - protein, 9 aa, synthetic construct
GGDGQDRLS

SEQ ID NO: 31607 - protein, 9 aa, synthetic construct
GGDGQDRLT

SEQ ID NO: 31608 - protein, 9 aa, synthetic construct
GGDGQDSAA

SEQ ID NO: 31609 - protein, 9 aa, synthetic construct
GGDGQDSAY

SEQ ID NO: 31610 - protein, 9 aa, synthetic construct
GGDGQDSID

SEQ ID NO: 31611 - protein, 9 aa, synthetic construct
GGDGQDSIN

SEQ ID NO: 31612 - protein, 9 aa, synthetic construct
GGDGQDSIS

SEQ ID NO: 31613 - protein, 9 aa, synthetic construct
GGDGQDTAL

SEQ ID NO: 31614 - protein, 9 aa, synthetic construct
GGDGQDQLD

SEQ ID NO: 31615 - protein, 9 aa, synthetic construct
GGDGQDNLD

SEQ ID NO: 31616 - protein, 9 aa, synthetic construct
GGDGQDNIN

SEQ ID NO: 31617 - protein, 9 aa, synthetic construct
GGDGQDNIG

SEQ ID NO: 31618 - protein, 9 aa, synthetic construct
GGDGQDHLY

SEQ ID NO: 31619 - protein, 9 aa, synthetic construct
GGDGQDIFK

SEQ ID NO: 31620 - protein, 9 aa, synthetic construct
GGDGQDIFR

SEQ ID NO: 31621 - protein, 9 aa, synthetic construct
GGDGQDIIL

SEQ ID NO: 31622 - protein, 9 aa, synthetic construct
GGDGQDILQ

SEQ ID NO: 31623 - protein, 9 aa, synthetic construct
GGDGQDILT

SEQ ID NO: 31624 - protein, 9 aa, synthetic construct
GGDGQDKLF

SEQ ID NO: 31625 - protein, 9 aa, synthetic construct
GGDGQDKLT

SEQ ID NO: 31626 - protein, 9 aa, synthetic construct
GGDGQDKLV

SEQ ID NO: 31627 - protein, 9 aa, synthetic construct
GGDGQDLAL

SEQ ID NO: 31628 - protein, 9 aa, synthetic construct
GGDGQDLIF

SEQ ID NO: 31629 - protein, 9 aa, synthetic construct
GGDGQDLIL

SEQ ID NO: 31630 - protein, 9 aa, synthetic construct
GGDGQDLIT

SEQ ID NO: 31631 - protein, 9 aa, synthetic construct
GGDGQDLLF

SEQ ID NO: 31632 - protein, 9 aa, synthetic construct
GGDGQDLLH

SEQ ID NO: 31633 - protein, 9 aa, synthetic construct
GGDGQDLLI

SEQ ID NO: 31634 - protein, 9 aa, synthetic construct
GGDGQDMLS

SEQ ID NO: 31635 - protein, 9 aa, synthetic construct
GGDGQDTAS

SEQ ID NO: 31636 - protein, 9 aa, synthetic construct
GGDGQDTAV

SEQ ID NO: 31637 - protein, 9 aa, synthetic construct
GGDGQDTIE

SEQ ID NO: 31638 - protein, 9 aa, synthetic construct
GGDGQDVLR

SEQ ID NO: 31639 - protein, 9 aa, synthetic construct
GGDGQDVLV

SEQ ID NO: 31640 - protein, 9 aa, synthetic construct
GGDGQDWLE

SEQ ID NO: 31641 - protein, 9 aa, synthetic construct
GGDGQDWLI

SEQ ID NO: 31642 - protein, 9 aa, synthetic construct
GGDGQDYIV

SEQ ID NO: 31643 - protein, 9 aa, synthetic construct
GGDGQDYLR

SEQ ID NO: 31644 - protein, 9 aa, synthetic construct
GGDGQDYLY

SEQ ID NO: 31645 - protein, 9 aa, synthetic construct
GGDGQDYMD

SEQ ID NO: 31646 - protein, 9 aa, synthetic construct
GGDGRDAFI

SEQ ID NO: 31647 - protein, 9 aa, synthetic construct
GGDGRDAFV

SEQ ID NO: 31648 - protein, 9 aa, synthetic construct
GGDGRDAIQ

SEQ ID NO: 31649 - protein, 9 aa, synthetic construct
GGDGRDALF

SEQ ID NO: 31650 - protein, 9 aa, synthetic construct
GGDGRDALH

SEQ ID NO: 31651 - protein, 9 aa, synthetic construct
GGDGRDALR

SEQ ID NO: 31652 - protein, 9 aa, synthetic construct
GGDGRDAMD

SEQ ID NO: 31653 - protein, 9 aa, synthetic construct
GGDGRDAVS

SEQ ID NO: 31654 - protein, 9 aa, synthetic construct
GGDGRDAYV

SEQ ID NO: 31655 - protein, 9 aa, synthetic construct
GGDGRDDFS

SEQ ID NO: 31656 - protein, 9 aa, synthetic construct
GGDGQDVLT

SEQ ID NO: 31657 - protein, 9 aa, synthetic construct
GGDGQDVLF

SEQ ID NO: 31658 - protein, 9 aa, synthetic construct
GGDGQDTIF

SEQ ID NO: 31659 - protein, 9 aa, synthetic construct
GGDGQDVLD

SEQ ID NO: 31660 - protein, 9 aa, synthetic construct
GGDGQDTIR

SEQ ID NO: 31661 - protein, 9 aa, synthetic construct
GGDGQDTIS

SEQ ID NO: 31662 - protein, 9 aa, synthetic construct
GGDGQDTIY

SEQ ID NO: 31663 - protein, 9 aa, synthetic construct
GGDGQDTLF

SEQ ID NO: 31664 - protein, 9 aa, synthetic construct
GGDGQDTLH

SEQ ID NO: 31665 - protein, 9 aa, synthetic construct
GGDGQDTLK

SEQ ID NO: 31666 - protein, 9 aa, synthetic construct
GGDGQDTLR

SEQ ID NO: 31667 - protein, 9 aa, synthetic construct
GGDGQDTLW

SEQ ID NO: 31668 - protein, 9 aa, synthetic construct
GGDGQDTMH

SEQ ID NO: 31669 - protein, 9 aa, synthetic construct
GGDGQDTMI

SEQ ID NO: 31670 - protein, 9 aa, synthetic construct
GGDGQDTVD

SEQ ID NO: 31671 - protein, 9 aa, synthetic construct
GGDGQDTVE

SEQ ID NO: 31672 - protein, 9 aa, synthetic construct
GGDGQDTVH

SEQ ID NO: 31673 - protein, 9 aa, synthetic construct
GGDGQDTYH

SEQ ID NO: 31674 - protein, 9 aa, synthetic construct
GGDGQDVAN

SEQ ID NO: 31675 - protein, 9 aa, synthetic construct
GGDGQDVIH

SEQ ID NO: 31676 - protein, 9 aa, synthetic construct
GGDGQDVIV

SEQ ID NO: 31677 - protein, 9 aa, synthetic construct
GGDGQDGID

SEQ ID NO: 31678 - protein, 9 aa, synthetic construct
GGDGQDFLV

SEQ ID NO: 31679 - protein, 9 aa, synthetic construct
GGDGQDFLR

SEQ ID NO: 31680 - protein, 9 aa, synthetic construct
GGDGNDYFS

SEQ ID NO: 31681 - protein, 9 aa, synthetic construct
GGDGNDYIL

SEQ ID NO: 31682 - protein, 9 aa, synthetic construct
GGDGNDYIM

SEQ ID NO: 31683 - protein, 9 aa, synthetic construct
GGDGNDYIR

SEQ ID NO: 31684 - protein, 9 aa, synthetic construct
GGDGNDYLG

SEQ ID NO: 31685 - protein, 9 aa, synthetic construct
GGDGNDYVH

SEQ ID NO: 31686 - protein, 9 aa, synthetic construct
GGDGNDYVR

SEQ ID NO: 31687 - protein, 9 aa, synthetic construct
GGDGNDYVS

SEQ ID NO: 31688 - protein, 9 aa, synthetic construct
GGDGNDYVV

SEQ ID NO: 31689 - protein, 9 aa, synthetic construct
GGDGPDFAN

SEQ ID NO: 31690 - protein, 9 aa, synthetic construct
GGDGPDFID

SEQ ID NO: 31691 - protein, 9 aa, synthetic construct
GGDGPDFLA

SEQ ID NO: 31692 - protein, 9 aa, synthetic construct
GGDGPDILK

SEQ ID NO: 31693 - protein, 9 aa, synthetic construct
GGDGPDILN

SEQ ID NO: 31694 - protein, 9 aa, synthetic construct
GGDGPDIMV

SEQ ID NO: 31695 - protein, 9 aa, synthetic construct
GGDGPDLAV

SEQ ID NO: 31696 - protein, 9 aa, synthetic construct
GGDGPDLIR

SEQ ID NO: 31697 - protein, 9 aa, synthetic construct
GGDGPDLIS

SEQ ID NO: 31698 - protein, 9 aa, synthetic construct
GGDGNDYII

SEQ ID NO: 31699 - protein, 9 aa, synthetic construct
GGDGNDYAS

SEQ ID NO: 31700 - protein, 9 aa, synthetic construct
GGDGPDLLS

SEQ ID NO: 31701 - protein, 9 aa, synthetic construct
GGDGNDYAR

SEQ ID NO: 31702 - protein, 9 aa, synthetic construct
GGDGNDVFR

SEQ ID NO: 31703 - protein, 9 aa, synthetic construct
GGDGNDVMF

SEQ ID NO: 31704 - protein, 9 aa, synthetic construct
GGDGNDVMI

SEQ ID NO: 31705 - protein, 9 aa, synthetic construct
GGDGNDVMM

SEQ ID NO: 31706 - protein, 9 aa, synthetic construct
GGDGNDVVV

SEQ ID NO: 31707 - protein, 9 aa, synthetic construct
GGDGNDVVW

SEQ ID NO: 31708 - protein, 9 aa, synthetic construct
GGDGNDVYE

SEQ ID NO: 31709 - protein, 9 aa, synthetic construct
GGDGNDVYS

SEQ ID NO: 31710 - protein, 9 aa, synthetic construct
GGDGNDWAL

SEQ ID NO: 31711 - protein, 9 aa, synthetic construct
GGDGNDWIL

SEQ ID NO: 31712 - protein, 9 aa, synthetic construct
GGDGNDWLG

SEQ ID NO: 31713 - protein, 9 aa, synthetic construct
GGDGNDWLQ

SEQ ID NO: 31714 - protein, 9 aa, synthetic construct
GGDGNDWLW

SEQ ID NO: 31715 - protein, 9 aa, synthetic construct
GGDGNDWMA

SEQ ID NO: 31716 - protein, 9 aa, synthetic construct
GGDGNDWMR

SEQ ID NO: 31717 - protein, 9 aa, synthetic construct
GGDGNDWMW

SEQ ID NO: 31718 - protein, 9 aa, synthetic construct
GGDGNDWVW

SEQ ID NO: 31719 - protein, 9 aa, synthetic construct
GGDGPDLLR

SEQ ID NO: 31720 - protein, 9 aa, synthetic construct
GGDGPDLLV

SEQ ID NO: 31721 - protein, 9 aa, synthetic construct
GGDGQDFIS

SEQ ID NO: 31722 - protein, 9 aa, synthetic construct
GGDGPDVLY

SEQ ID NO: 31723 - protein, 9 aa, synthetic construct
GGDGPDYLI

SEQ ID NO: 31724 - protein, 9 aa, synthetic construct
GGDGQDAAD

SEQ ID NO: 31725 - protein, 9 aa, synthetic construct
GGDGQDALA

SEQ ID NO: 31726 - protein, 9 aa, synthetic construct
GGDGQDALS

SEQ ID NO: 31727 - protein, 9 aa, synthetic construct
GGDGQDALY

SEQ ID NO: 31728 - protein, 9 aa, synthetic construct
GGDGQDAME

SEQ ID NO: 31729 - protein, 9 aa, synthetic construct
GGDGQDDID

SEQ ID NO: 31730 - protein, 9 aa, synthetic construct
GGDGQDDLD

SEQ ID NO: 31731 - protein, 9 aa, synthetic construct
GGDGQDDLK

SEQ ID NO: 31732 - protein, 9 aa, synthetic construct
GGDGQDEAT

SEQ ID NO: 31733 - protein, 9 aa, synthetic construct
GGDGQDELH

SEQ ID NO: 31734 - protein, 9 aa, synthetic construct
GGDGQDELL

SEQ ID NO: 31735 - protein, 9 aa, synthetic construct
GGDGQDELS

SEQ ID NO: 31736 - protein, 9 aa, synthetic construct
GGDGQDELW

SEQ ID NO: 31737 - protein, 9 aa, synthetic construct
GGDGQDFAM

SEQ ID NO: 31738 - protein, 9 aa, synthetic construct
GGDGQDFIN

SEQ ID NO: 31739 - protein, 9 aa, synthetic construct
GGDGQDFIR

SEQ ID NO: 31740 - protein, 9 aa, synthetic construct
GGDGPDWLA

SEQ ID NO: 31741 - protein, 9 aa, synthetic construct
GGDGPDVLI

SEQ ID NO: 31742 - protein, 9 aa, synthetic construct
GGDGPDLMF

SEQ ID NO: 31743 - protein, 9 aa, synthetic construct
GGDGPDVIL

SEQ ID NO: 31744 - protein, 9 aa, synthetic construct
GGDGPDLMQ

SEQ ID NO: 31745 - protein, 9 aa, synthetic construct
GGDGPDNIE

SEQ ID NO: 31746 - protein, 9 aa, synthetic construct
GGDGPDQIS

SEQ ID NO: 31747 - protein, 9 aa, synthetic construct
GGDGPDQIY

SEQ ID NO: 31748 - protein, 9 aa, synthetic construct
GGDGPDQLE

SEQ ID NO: 31749 - protein, 9 aa, synthetic construct
GGDGPDRFE

SEQ ID NO: 31750 - protein, 9 aa, synthetic construct
GGDGPDRIE

SEQ ID NO: 31751 - protein, 9 aa, synthetic construct
GGDGPDRLR

SEQ ID NO: 31752 - protein, 9 aa, synthetic construct
GGDGPDSLD

SEQ ID NO: 31753 - protein, 9 aa, synthetic construct
GGDGPDTFR

SEQ ID NO: 31754 - protein, 9 aa, synthetic construct
GGDGPDTIV

SEQ ID NO: 31755 - protein, 9 aa, synthetic construct
GGDGPDTIY

SEQ ID NO: 31756 - protein, 9 aa, synthetic construct
GGDGPDTLD

SEQ ID NO: 31757 - protein, 9 aa, synthetic construct
GGDGPDTLF

SEQ ID NO: 31758 - protein, 9 aa, synthetic construct
GGDGPDTLM

SEQ ID NO: 31759 - protein, 9 aa, synthetic construct
GGDGPDTLN

SEQ ID NO: 31760 - protein, 9 aa, synthetic construct
GGDGPDTLY

SEQ ID NO: 31761 - protein, 9 aa, synthetic construct
GGDGNDGID

SEQ ID NO: 31762 - protein, 9 aa, synthetic construct
GGDGNDGFA

SEQ ID NO: 31763 - protein, 9 aa, synthetic construct
GGDGNDFYI

SEQ ID NO: 31764 - protein, 9 aa, synthetic construct
GGDGKDTIN

SEQ ID NO: 31765 - protein, 9 aa, synthetic construct
GGDGKDSLA

SEQ ID NO: 31766 - protein, 9 aa, synthetic construct
GGDGKDSLR

SEQ ID NO: 31767 - protein, 9 aa, synthetic construct
GGDGKDSVY

SEQ ID NO: 31768 - protein, 9 aa, synthetic construct
GGDGKDSYL

SEQ ID NO: 31769 - protein, 9 aa, synthetic construct
GGDGKDTAS

SEQ ID NO: 31770 - protein, 9 aa, synthetic construct
GGDGKDTFI

SEQ ID NO: 31771 - protein, 9 aa, synthetic construct
GGDGKDTFV

SEQ ID NO: 31772 - protein, 9 aa, synthetic construct
GGDGKDTIH

SEQ ID NO: 31773 - protein, 9 aa, synthetic construct
GGDGKDTLA

SEQ ID NO: 31774 - protein, 9 aa, synthetic construct
GGDGNDFVQ

SEQ ID NO: 31775 - protein, 9 aa, synthetic construct
GGDGKDTLF

SEQ ID NO: 31776 - protein, 9 aa, synthetic construct
GGDGKDTLH

SEQ ID NO: 31777 - protein, 9 aa, synthetic construct
GGDGKDTVR

SEQ ID NO: 31778 - protein, 9 aa, synthetic construct
GGDGKDTVS

SEQ ID NO: 31779 - protein, 9 aa, synthetic construct
GGDGKDVAS

SEQ ID NO: 31780 - protein, 9 aa, synthetic construct
GGDGKDVFE

SEQ ID NO: 31781 - protein, 9 aa, synthetic construct
GGDGKDVFM

SEQ ID NO: 31782 - protein, 9 aa, synthetic construct
GGDGKDVID

SEQ ID NO: 31783 - protein, 9 aa, synthetic construct
GGDGKDSIK

SEQ ID NO: 31784 - protein, 9 aa, synthetic construct
GGDGKDRMT

SEQ ID NO: 31785 - protein, 9 aa, synthetic construct
GGDGKDRLY

SEQ ID NO: 31786 - protein, 9 aa, synthetic construct
GGDGKDRLI

SEQ ID NO: 31787 - protein, 9 aa, synthetic construct
GGDGKDMLI

SEQ ID NO: 31788 - protein, 9 aa, synthetic construct
GGDGKDMLN

SEQ ID NO: 31789 - protein, 9 aa, synthetic construct
GGDGKDMVV

SEQ ID NO: 31790 - protein, 9 aa, synthetic construct
GGDGKDNIF

SEQ ID NO: 31791 - protein, 9 aa, synthetic construct
GGDGKDNIS

SEQ ID NO: 31792 - protein, 9 aa, synthetic construct
GGDGKDNLF

SEQ ID NO: 31793 - protein, 9 aa, synthetic construct
GGDGKDNLK

SEQ ID NO: 31794 - protein, 9 aa, synthetic construct
GGDGKDNLQ

SEQ ID NO: 31795 - protein, 9 aa, synthetic construct
GGDGKDNVS

SEQ ID NO: 31796 - protein, 9 aa, synthetic construct
GGDGKDQIA

SEQ ID NO: 31797 - protein, 9 aa, synthetic construct
GGDGKDQLR

SEQ ID NO: 31798 - protein, 9 aa, synthetic construct
GGDGKDQLS

SEQ ID NO: 31799 - protein, 9 aa, synthetic construct
GGDGKDQLT

SEQ ID NO: 31800 - protein, 9 aa, synthetic construct
GGDGKDRID

SEQ ID NO: 31801 - protein, 9 aa, synthetic construct
GGDGKDRIE

SEQ ID NO: 31802 - protein, 9 aa, synthetic construct
GGDGKDRLA

SEQ ID NO: 31803 - protein, 9 aa, synthetic construct
GGDGKDRLD

SEQ ID NO: 31804 - protein, 9 aa, synthetic construct
GGDGKDVIE

SEQ ID NO: 31805 - protein, 9 aa, synthetic construct
GGDGKDVIV

SEQ ID NO: 31806 - protein, 9 aa, synthetic construct
GGDGKDVIW

SEQ ID NO: 31807 - protein, 9 aa, synthetic construct
GGDGLDELH

SEQ ID NO: 31808 - protein, 9 aa, synthetic construct
GGDGLDELY

SEQ ID NO: 31809 - protein, 9 aa, synthetic construct
GGDGLDFAF

SEQ ID NO: 31810 - protein, 9 aa, synthetic construct
GGDGLDFIR

SEQ ID NO: 31811 - protein, 9 aa, synthetic construct
GGDGLDFLA

SEQ ID NO: 31812 - protein, 9 aa, synthetic construct
GGDGLDFLF

SEQ ID NO: 31813 - protein, 9 aa, synthetic construct
GGDGLDFVS

SEQ ID NO: 31814 - protein, 9 aa, synthetic construct
GGDGLDHLD

SEQ ID NO: 31815 - protein, 9 aa, synthetic construct
GGDGLDIAD

SEQ ID NO: 31816 - protein, 9 aa, synthetic construct
GGDGLDIAF

SEQ ID NO: 31817 - protein, 9 aa, synthetic construct
GGDGLDIAS

SEQ ID NO: 31818 - protein, 9 aa, synthetic construct
GGDGLDIID

SEQ ID NO: 31819 - protein, 9 aa, synthetic construct
GGDGLDILL

SEQ ID NO: 31820 - protein, 9 aa, synthetic construct
GGDGLDILN

SEQ ID NO: 31821 - protein, 9 aa, synthetic construct
GGDGLDILS

SEQ ID NO: 31822 - protein, 9 aa, synthetic construct
GGDGLDIMT

SEQ ID NO: 31823 - protein, 9 aa, synthetic construct
GGDGLDIVS

SEQ ID NO: 31824 - protein, 9 aa, synthetic construct
GGDGLDKFV

SEQ ID NO: 31825 - protein, 9 aa, synthetic construct
GGDGLDELT

SEQ ID NO: 31826 - protein, 9 aa, synthetic construct
GGDGLDELF

SEQ ID NO: 31827 - protein, 9 aa, synthetic construct
GGDGKDVLH

SEQ ID NO: 31828 - protein, 9 aa, synthetic construct
GGDGLDEIN

SEQ ID NO: 31829 - protein, 9 aa, synthetic construct
GGDGKDVLI

SEQ ID NO: 31830 - protein, 9 aa, synthetic construct
GGDGKDVLL

SEQ ID NO: 31831 - protein, 9 aa, synthetic construct
GGDGKDVVR

SEQ ID NO: 31832 - protein, 9 aa, synthetic construct
GGDGKDWIN

SEQ ID NO: 31833 - protein, 9 aa, synthetic construct
GGDGKDWLD

SEQ ID NO: 31834 - protein, 9 aa, synthetic construct
GGDGKDWLF

SEQ ID NO: 31835 - protein, 9 aa, synthetic construct
GGDGKDWLH

SEQ ID NO: 31836 - protein, 9 aa, synthetic construct
GGDGKDWMG

SEQ ID NO: 31837 - protein, 9 aa, synthetic construct
GGDGKDYLH

SEQ ID NO: 31838 - protein, 9 aa, synthetic construct
GGDGKDYLN

SEQ ID NO: 31839 - protein, 9 aa, synthetic construct
GGDGKDYLR

SEQ ID NO: 31840 - protein, 9 aa, synthetic construct
GGDGLDAIS

SEQ ID NO: 31841 - protein, 9 aa, synthetic construct
GGDGLDALF

SEQ ID NO: 31842 - protein, 9 aa, synthetic construct
GGDGLDDID

SEQ ID NO: 31843 - protein, 9 aa, synthetic construct
GGDGLDDLV

SEQ ID NO: 31844 - protein, 9 aa, synthetic construct
GGDGLDDLY

SEQ ID NO: 31845 - protein, 9 aa, synthetic construct
GGDGLDEFD

SEQ ID NO: 31846 - protein, 9 aa, synthetic construct
GGDGKDMLA

SEQ ID NO: 31847 - protein, 9 aa, synthetic construct
GGDGKDLVS

SEQ ID NO: 31848 - protein, 9 aa, synthetic construct
GGDGKDLLK

SEQ ID NO: 31849 - protein, 9 aa, synthetic construct
GGDGIDVAS

SEQ ID NO: 31850 - protein, 9 aa, synthetic construct
GGDGIDVFG

SEQ ID NO: 31851 - protein, 9 aa, synthetic construct
GGDGIDVIE

SEQ ID NO: 31852 - protein, 9 aa, synthetic construct
GGDGIDVIN

SEQ ID NO: 31853 - protein, 9 aa, synthetic construct
GGDGIDVLF

SEQ ID NO: 31854 - protein, 9 aa, synthetic construct
GGDGIDVLN

SEQ ID NO: 31855 - protein, 9 aa, synthetic construct
GGDGIDVLT

SEQ ID NO: 31856 - protein, 9 aa, synthetic construct
GGDGIDVLV

SEQ ID NO: 31857 - protein, 9 aa, synthetic construct
GGDGIDVML

SEQ ID NO: 31858 - protein, 9 aa, synthetic construct
GGDGIDVMN

SEQ ID NO: 31859 - protein, 9 aa, synthetic construct
GGDGIDWLE

SEQ ID NO: 31860 - protein, 9 aa, synthetic construct
GGDGIDWLH

SEQ ID NO: 31861 - protein, 9 aa, synthetic construct
GGDGIDWLI

SEQ ID NO: 31862 - protein, 9 aa, synthetic construct
GGDGIDWLQ

SEQ ID NO: 31863 - protein, 9 aa, synthetic construct
GGDGIDWVR

SEQ ID NO: 31864 - protein, 9 aa, synthetic construct
GGDGIDWVS

SEQ ID NO: 31865 - protein, 9 aa, synthetic construct
GGDGIDYLE

SEQ ID NO: 31866 - protein, 9 aa, synthetic construct
GGDGIDYLF

SEQ ID NO: 31867 - protein, 9 aa, synthetic construct
GGDGIDVAV

SEQ ID NO: 31868 - protein, 9 aa, synthetic construct
GGDGIDVAD

SEQ ID NO: 31869 - protein, 9 aa, synthetic construct
GGDGKDALF

SEQ ID NO: 31870 - protein, 9 aa, synthetic construct
GGDGIDVAA

SEQ ID NO: 31871 - protein, 9 aa, synthetic construct
GGDGIDTAE

SEQ ID NO: 31872 - protein, 9 aa, synthetic construct
GGDGIDTAG

SEQ ID NO: 31873 - protein, 9 aa, synthetic construct
GGDGIDTAL

SEQ ID NO: 31874 - protein, 9 aa, synthetic construct
GGDGIDTAP

SEQ ID NO: 31875 - protein, 9 aa, synthetic construct
GGDGIDTAY

SEQ ID NO: 31876 - protein, 9 aa, synthetic construct
GGDGIDTFV

SEQ ID NO: 31877 - protein, 9 aa, synthetic construct
GGDGIDTID

SEQ ID NO: 31878 - protein, 9 aa, synthetic construct
GGDGIDTIF

SEQ ID NO: 31879 - protein, 9 aa, synthetic construct
GGDGIDTIK

SEQ ID NO: 31880 - protein, 9 aa, synthetic construct
GGDGIDTIL

SEQ ID NO: 31881 - protein, 9 aa, synthetic construct
GGDGIDTMI

SEQ ID NO: 31882 - protein, 9 aa, synthetic construct
GGDGIDTMK

SEQ ID NO: 31883 - protein, 9 aa, synthetic construct
GGDGIDTMT

SEQ ID NO: 31884 - protein, 9 aa, synthetic construct
GGDGIDTVI

SEQ ID NO: 31885 - protein, 9 aa, synthetic construct
GGDGIDTVR

SEQ ID NO: 31886 - protein, 9 aa, synthetic construct
GGDGIDTVY

SEQ ID NO: 31887 - protein, 9 aa, synthetic construct
GGDGIDTYY

SEQ ID NO: 31888 - protein, 9 aa, synthetic construct
GGDGIDYLS

SEQ ID NO: 31889 - protein, 9 aa, synthetic construct
GGDGKDALI

SEQ ID NO: 31890 - protein, 9 aa, synthetic construct
GGDGKDLLF

SEQ ID NO: 31891 - protein, 9 aa, synthetic construct
GGDGKDIIK

SEQ ID NO: 31892 - protein, 9 aa, synthetic construct
GGDGKDIIY

SEQ ID NO: 31893 - protein, 9 aa, synthetic construct
GGDGKDILI

SEQ ID NO: 31894 - protein, 9 aa, synthetic construct
GGDGKDILL

SEQ ID NO: 31895 - protein, 9 aa, synthetic construct
GGDGKDILY

SEQ ID NO: 31896 - protein, 9 aa, synthetic construct
GGDGKDKIE

SEQ ID NO: 31897 - protein, 9 aa, synthetic construct
GGDGKDKIF

SEQ ID NO: 31898 - protein, 9 aa, synthetic construct
GGDGKDKIG

SEQ ID NO: 31899 - protein, 9 aa, synthetic construct
GGDGKDKIS

SEQ ID NO: 31900 - protein, 9 aa, synthetic construct
GGDGKDKLE

SEQ ID NO: 31901 - protein, 9 aa, synthetic construct
GGDGKDKLF

SEQ ID NO: 31902 - protein, 9 aa, synthetic construct
GGDGKDKLT

SEQ ID NO: 31903 - protein, 9 aa, synthetic construct
GGDGKDKLV

SEQ ID NO: 31904 - protein, 9 aa, synthetic construct
GGDGKDKLY

SEQ ID NO: 31905 - protein, 9 aa, synthetic construct
GGDGKDKVF

SEQ ID NO: 31906 - protein, 9 aa, synthetic construct
GGDGKDKVY

SEQ ID NO: 31907 - protein, 9 aa, synthetic construct
GGDGKDLFK

SEQ ID NO: 31908 - protein, 9 aa, synthetic construct
GGDGKDLIR

SEQ ID NO: 31909 - protein, 9 aa, synthetic construct
GGDGKDIIV

SEQ ID NO: 31910 - protein, 9 aa, synthetic construct
GGDGKDIFR

SEQ ID NO: 31911 - protein, 9 aa, synthetic construct
GGDGKDALL

SEQ ID NO: 31912 - protein, 9 aa, synthetic construct
GGDGKDIFL

SEQ ID NO: 31913 - protein, 9 aa, synthetic construct
GGDGKDAMR

SEQ ID NO: 31914 - protein, 9 aa, synthetic construct
GGDGKDDLH

SEQ ID NO: 31915 - protein, 9 aa, synthetic construct
GGDGKDEAQ

SEQ ID NO: 31916 - protein, 9 aa, synthetic construct
GGDGKDEIY

SEQ ID NO: 31917 - protein, 9 aa, synthetic construct
GGDGKDELE

SEQ ID NO: 31918 - protein, 9 aa, synthetic construct
GGDGKDELH

SEQ ID NO: 31919 - protein, 9 aa, synthetic construct
GGDGKDELY

SEQ ID NO: 31920 - protein, 9 aa, synthetic construct
GGDGKDEMF

SEQ ID NO: 31921 - protein, 9 aa, synthetic construct
GGDGKDFID

SEQ ID NO: 31922 - protein, 9 aa, synthetic construct
GGDGKDFLD

SEQ ID NO: 31923 - protein, 9 aa, synthetic construct
GGDGKDFLH

SEQ ID NO: 31924 - protein, 9 aa, synthetic construct
GGDGKDFLS

SEQ ID NO: 31925 - protein, 9 aa, synthetic construct
GGDGKDFMD

SEQ ID NO: 31926 - protein, 9 aa, synthetic construct
GGDGKDFMK

SEQ ID NO: 31927 - protein, 9 aa, synthetic construct
GGDGKDGLF

SEQ ID NO: 31928 - protein, 9 aa, synthetic construct
GGDGKDHIN

SEQ ID NO: 31929 - protein, 9 aa, synthetic construct
GGDGKDHLT

SEQ ID NO: 31930 - protein, 9 aa, synthetic construct
GGDGLDLIF

SEQ ID NO: 31931 - protein, 9 aa, synthetic construct
GGDGLDLLA

SEQ ID NO: 31932 - protein, 9 aa, synthetic construct
GGDGLDLLI

SEQ ID NO: 31933 - protein, 9 aa, synthetic construct
GGDGNDAMA

SEQ ID NO: 31934 - protein, 9 aa, synthetic construct
GGDGNDAMS

SEQ ID NO: 31935 - protein, 9 aa, synthetic construct
GGDGNDAMW

SEQ ID NO: 31936 - protein, 9 aa, synthetic construct
GGDGNDAVL

SEQ ID NO: 31937 - protein, 9 aa, synthetic construct
GGDGNDAVS

SEQ ID NO: 31938 - protein, 9 aa, synthetic construct
GGDGNDAVT

SEQ ID NO: 31939 - protein, 9 aa, synthetic construct
GGDGNDAYI

SEQ ID NO: 31940 - protein, 9 aa, synthetic construct
GGDGNDCID

SEQ ID NO: 31941 - protein, 9 aa, synthetic construct
GGDGNDCLT

SEQ ID NO: 31942 - protein, 9 aa, synthetic construct
GGDGNDCLW

SEQ ID NO: 31943 - protein, 9 aa, synthetic construct
GGDGNDCYV

SEQ ID NO: 31944 - protein, 9 aa, synthetic construct
GGDGNDDIL

SEQ ID NO: 31945 - protein, 9 aa, synthetic construct
GGDGNDDIT

SEQ ID NO: 31946 - protein, 9 aa, synthetic construct
GGDGNDDIV

SEQ ID NO: 31947 - protein, 9 aa, synthetic construct
GGDGNDDLL

SEQ ID NO: 31948 - protein, 9 aa, synthetic construct
GGDGNDDLN

SEQ ID NO: 31949 - protein, 9 aa, synthetic construct
GGDGNDDLT

SEQ ID NO: 31950 - protein, 9 aa, synthetic construct
GGDGNDDLY

SEQ ID NO: 31951 - protein, 9 aa, synthetic construct
GGDGNDAMD

SEQ ID NO: 31952 - protein, 9 aa, synthetic construct
GGDGNDALK

SEQ ID NO: 31953 - protein, 9 aa, synthetic construct
GGDGNDDMG

SEQ ID NO: 31954 - protein, 9 aa, synthetic construct
GGDGNDAIV

SEQ ID NO: 31955 - protein, 9 aa, synthetic construct
GGDGMDTID

SEQ ID NO: 31956 - protein, 9 aa, synthetic construct
GGDGMDTIV

SEQ ID NO: 31957 - protein, 9 aa, synthetic construct
GGDGMDTLD

SEQ ID NO: 31958 - protein, 9 aa, synthetic construct
GGDGMDTLH

SEQ ID NO: 31959 - protein, 9 aa, synthetic construct
GGDGMDTLN

SEQ ID NO: 31960 - protein, 9 aa, synthetic construct
GGDGMDTLS

SEQ ID NO: 31961 - protein, 9 aa, synthetic construct
GGDGMDTVD

SEQ ID NO: 31962 - protein, 9 aa, synthetic construct
GGDGMDTVS

SEQ ID NO: 31963 - protein, 9 aa, synthetic construct
GGDGMDVLD

SEQ ID NO: 31964 - protein, 9 aa, synthetic construct
GGDGMDVLV

SEQ ID NO: 31965 - protein, 9 aa, synthetic construct
GGDGMDVVN

SEQ ID NO: 31966 - protein, 9 aa, synthetic construct
GGDGMDYAV

SEQ ID NO: 31967 - protein, 9 aa, synthetic construct
GGDGMDYVY

SEQ ID NO: 31968 - protein, 9 aa, synthetic construct
GGDGNDAAA

SEQ ID NO: 31969 - protein, 9 aa, synthetic construct
GGDGNDAAY

SEQ ID NO: 31970 - protein, 9 aa, synthetic construct
GGDGNDAII

SEQ ID NO: 31971 - protein, 9 aa, synthetic construct
GGDGNDAIQ

SEQ ID NO: 31972 - protein, 9 aa, synthetic construct
GGDGNDDMD

SEQ ID NO: 31973 - protein, 9 aa, synthetic construct
GGDGNDDMR

SEQ ID NO: 31974 - protein, 9 aa, synthetic construct
GGDGMDTFI

SEQ ID NO: 31975 - protein, 9 aa, synthetic construct
GGDGNDEMT

SEQ ID NO: 31976 - protein, 9 aa, synthetic construct
GGDGNDEVW

SEQ ID NO: 31977 - protein, 9 aa, synthetic construct
GGDGNDEVY

SEQ ID NO: 31978 - protein, 9 aa, synthetic construct
GGDGNDFAF

SEQ ID NO: 31979 - protein, 9 aa, synthetic construct
GGDGNDFFY

SEQ ID NO: 31980 - protein, 9 aa, synthetic construct
GGDGNDFIE

SEQ ID NO: 31981 - protein, 9 aa, synthetic construct
GGDGNDFIK

SEQ ID NO: 31982 - protein, 9 aa, synthetic construct
GGDGNDFLE

SEQ ID NO: 31983 - protein, 9 aa, synthetic construct
GGDGNDFLK

SEQ ID NO: 31984 - protein, 9 aa, synthetic construct
GGDGNDFLM

SEQ ID NO: 31985 - protein, 9 aa, synthetic construct
GGDGNDFLW

SEQ ID NO: 31986 - protein, 9 aa, synthetic construct
GGDGNDFMD

SEQ ID NO: 31987 - protein, 9 aa, synthetic construct
GGDGNDFMN

SEQ ID NO: 31988 - protein, 9 aa, synthetic construct
GGDGNDFMS

SEQ ID NO: 31989 - protein, 9 aa, synthetic construct
GGDGNDFMV

SEQ ID NO: 31990 - protein, 9 aa, synthetic construct
GGDGNDFVE

SEQ ID NO: 31991 - protein, 9 aa, synthetic construct
GGDGNDFVI

SEQ ID NO: 31992 - protein, 9 aa, synthetic construct
GGDGNDFVK

SEQ ID NO: 31993 - protein, 9 aa, synthetic construct
GGDGNDEVA

SEQ ID NO: 31994 - protein, 9 aa, synthetic construct
GGDGNDEMS

SEQ ID NO: 31995 - protein, 9 aa, synthetic construct
GGDGNDDMS

SEQ ID NO: 31996 - protein, 9 aa, synthetic construct
GGDGNDEMQ

SEQ ID NO: 31997 - protein, 9 aa, synthetic construct
GGDGNDDVD

SEQ ID NO: 31998 - protein, 9 aa, synthetic construct
GGDGNDDYR

SEQ ID NO: 31999 - protein, 9 aa, synthetic construct
GGDGNDEAG

SEQ ID NO: 32000 - protein, 9 aa, synthetic construct
GGDGNDEAN

SEQ ID NO: 32001 - protein, 9 aa, synthetic construct
GGDGNDEAR

SEQ ID NO: 32002 - protein, 9 aa, synthetic construct
GGDGNDEFI

SEQ ID NO: 32003 - protein, 9 aa, synthetic construct
GGDGNDEFK

SEQ ID NO: 32004 - protein, 9 aa, synthetic construct
GGDGNDEFT

SEQ ID NO: 32005 - protein, 9 aa, synthetic construct
GGDGNDEIE

SEQ ID NO: 32006 - protein, 9 aa, synthetic construct
GGDGNDEIF

SEQ ID NO: 32007 - protein, 9 aa, synthetic construct
GGDGNDEIG

SEQ ID NO: 32008 - protein, 9 aa, synthetic construct
GGDGNDEIN

SEQ ID NO: 32009 - protein, 9 aa, synthetic construct
GGDGNDEIT

SEQ ID NO: 32010 - protein, 9 aa, synthetic construct
GGDGNDEIW

SEQ ID NO: 32011 - protein, 9 aa, synthetic construct
GGDGNDELE

SEQ ID NO: 32012 - protein, 9 aa, synthetic construct
GGDGNDELQ

SEQ ID NO: 32013 - protein, 9 aa, synthetic construct
GGDGNDEMF

SEQ ID NO: 32014 - protein, 9 aa, synthetic construct
GGDGMDTFR

SEQ ID NO: 32015 - protein, 9 aa, synthetic construct
GGDGMDTAV

SEQ ID NO: 32016 - protein, 9 aa, synthetic construct
GGDGLDLLV

SEQ ID NO: 32017 - protein, 9 aa, synthetic construct
GGDGLDSIV

SEQ ID NO: 32018 - protein, 9 aa, synthetic construct
GGDGLDSLE

SEQ ID NO: 32019 - protein, 9 aa, synthetic construct
GGDGLDSLF

SEQ ID NO: 32020 - protein, 9 aa, synthetic construct
GGDGLDSLI

SEQ ID NO: 32021 - protein, 9 aa, synthetic construct
GGDGLDSLN

SEQ ID NO: 32022 - protein, 9 aa, synthetic construct
GGDGLDSLT

SEQ ID NO: 32023 - protein, 9 aa, synthetic construct
GGDGLDTAY

SEQ ID NO: 32024 - protein, 9 aa, synthetic construct
GGDGLDTFN

SEQ ID NO: 32025 - protein, 9 aa, synthetic construct
GGDGLDTFR

SEQ ID NO: 32026 - protein, 9 aa, synthetic construct
GGDGLDTIE

SEQ ID NO: 32027 - protein, 9 aa, synthetic construct
GGDGLDTIF

SEQ ID NO: 32028 - protein, 9 aa, synthetic construct
GGDGLDTIY

SEQ ID NO: 32029 - protein, 9 aa, synthetic construct
GGDGLDTLK

SEQ ID NO: 32030 - protein, 9 aa, synthetic construct
GGDGLDTLM

SEQ ID NO: 32031 - protein, 9 aa, synthetic construct
GGDGLDTLQ

SEQ ID NO: 32032 - protein, 9 aa, synthetic construct
GGDGLDTLW

SEQ ID NO: 32033 - protein, 9 aa, synthetic construct
GGDGLDTMN

SEQ ID NO: 32034 - protein, 9 aa, synthetic construct
GGDGLDTVS

SEQ ID NO: 32035 - protein, 9 aa, synthetic construct
GGDGLDSIW

SEQ ID NO: 32036 - protein, 9 aa, synthetic construct
GGDGLDSII

SEQ ID NO: 32037 - protein, 9 aa, synthetic construct
GGDGLDVFV

SEQ ID NO: 32038 - protein, 9 aa, synthetic construct
GGDGLDSFS

SEQ ID NO: 32039 - protein, 9 aa, synthetic construct
GGDGLDLLY

SEQ ID NO: 32040 - protein, 9 aa, synthetic construct
GGDGLDLMI

SEQ ID NO: 32041 - protein, 9 aa, synthetic construct
GGDGLDLVF

SEQ ID NO: 32042 - protein, 9 aa, synthetic construct
GGDGLDMAS

SEQ ID NO: 32043 - protein, 9 aa, synthetic construct
GGDGLDNLF

SEQ ID NO: 32044 - protein, 9 aa, synthetic construct
GGDGLDNLQ

SEQ ID NO: 32045 - protein, 9 aa, synthetic construct
GGDGLDQIY

SEQ ID NO: 32046 - protein, 9 aa, synthetic construct
GGDGLDQLE

SEQ ID NO: 32047 - protein, 9 aa, synthetic construct
GGDGLDQLT

SEQ ID NO: 32048 - protein, 9 aa, synthetic construct
GGDGLDRAT

SEQ ID NO: 32049 - protein, 9 aa, synthetic construct
GGDGLDRFL

SEQ ID NO: 32050 - protein, 9 aa, synthetic construct
GGDGLDRIE

SEQ ID NO: 32051 - protein, 9 aa, synthetic construct
GGDGLDRIV

SEQ ID NO: 32052 - protein, 9 aa, synthetic construct
GGDGLDRLD

SEQ ID NO: 32053 - protein, 9 aa, synthetic construct
GGDGLDRLL

SEQ ID NO: 32054 - protein, 9 aa, synthetic construct
GGDGLDRLM

SEQ ID NO: 32055 - protein, 9 aa, synthetic construct
GGDGLDRLV

SEQ ID NO: 32056 - protein, 9 aa, synthetic construct
GGDGLDVAE

SEQ ID NO: 32057 - protein, 9 aa, synthetic construct
GGDGLDVID

SEQ ID NO: 32058 - protein, 9 aa, synthetic construct
GGDGMDSLS

SEQ ID NO: 32059 - protein, 9 aa, synthetic construct
GGDGMDFIM

SEQ ID NO: 32060 - protein, 9 aa, synthetic construct
GGDGMDIFK

SEQ ID NO: 32061 - protein, 9 aa, synthetic construct
GGDGMDILE

SEQ ID NO: 32062 - protein, 9 aa, synthetic construct
GGDGMDILI

SEQ ID NO: 32063 - protein, 9 aa, synthetic construct
GGDGMDKMD

SEQ ID NO: 32064 - protein, 9 aa, synthetic construct
GGDGMDLIH

SEQ ID NO: 32065 - protein, 9 aa, synthetic construct
GGDGMDLIT

SEQ ID NO: 32066 - protein, 9 aa, synthetic construct
GGDGMDLLF

SEQ ID NO: 32067 - protein, 9 aa, synthetic construct
GGDGMDLLI

SEQ ID NO: 32068 - protein, 9 aa, synthetic construct
GGDGMDLLS

SEQ ID NO: 32069 - protein, 9 aa, synthetic construct
GGDGMDLLV

SEQ ID NO: 32070 - protein, 9 aa, synthetic construct
GGDGMDMID

SEQ ID NO: 32071 - protein, 9 aa, synthetic construct
GGDGMDMLA

SEQ ID NO: 32072 - protein, 9 aa, synthetic construct
GGDGMDMLI

SEQ ID NO: 32073 - protein, 9 aa, synthetic construct
GGDGMDRID

SEQ ID NO: 32074 - protein, 9 aa, synthetic construct
GGDGMDRIF

SEQ ID NO: 32075 - protein, 9 aa, synthetic construct
GGDGMDSLD

SEQ ID NO: 32076 - protein, 9 aa, synthetic construct
GGDGMDSLN

SEQ ID NO: 32077 - protein, 9 aa, synthetic construct
GGDGMDFLV

SEQ ID NO: 32078 - protein, 9 aa, synthetic construct
GGDGMDELS

SEQ ID NO: 32079 - protein, 9 aa, synthetic construct
GGDGLDVIE

SEQ ID NO: 32080 - protein, 9 aa, synthetic construct
GGDGMDCLV

SEQ ID NO: 32081 - protein, 9 aa, synthetic construct
GGDGLDVIV

SEQ ID NO: 32082 - protein, 9 aa, synthetic construct
GGDGLDVIY

SEQ ID NO: 32083 - protein, 9 aa, synthetic construct
GGDGLDVLD

SEQ ID NO: 32084 - protein, 9 aa, synthetic construct
GGDGLDVLI

SEQ ID NO: 32085 - protein, 9 aa, synthetic construct
GGDGLDVLQ

SEQ ID NO: 32086 - protein, 9 aa, synthetic construct
GGDGLDVLS

SEQ ID NO: 32087 - protein, 9 aa, synthetic construct
GGDGLDVMM

SEQ ID NO: 32088 - protein, 9 aa, synthetic construct
GGDGLDVMY

SEQ ID NO: 32089 - protein, 9 aa, synthetic construct
GGDGLDVVS

SEQ ID NO: 32090 - protein, 9 aa, synthetic construct
GGDGLDVYR

SEQ ID NO: 32091 - protein, 9 aa, synthetic construct
GGDGLDWAA

SEQ ID NO: 32092 - protein, 9 aa, synthetic construct
GGDGLDWAS

SEQ ID NO: 32093 - protein, 9 aa, synthetic construct
GGDGLDWLI

SEQ ID NO: 32094 - protein, 9 aa, synthetic construct
GGDGLDYLY

SEQ ID NO: 32095 - protein, 9 aa, synthetic construct
GGDGLDYMD

SEQ ID NO: 32096 - protein, 9 aa, synthetic construct
GGDGLDYVD

SEQ ID NO: 32097 - protein, 9 aa, synthetic construct
GGDGMDAIS

SEQ ID NO: 32098 - protein, 9 aa, synthetic construct
GGDGRDDIS

SEQ ID NO: 32099 - protein, 9 aa, synthetic construct
GGDGRDDLD

SEQ ID NO: 32100 - protein, 9 aa, synthetic construct
GGDGIDSLY

SEQ ID NO: 32101 - protein, 9 aa, synthetic construct
GGDGVDFLD

SEQ ID NO: 32102 - protein, 9 aa, synthetic construct
GGDGVDEAD

SEQ ID NO: 32103 - protein, 9 aa, synthetic construct
GGDGVDEIH

SEQ ID NO: 32104 - protein, 9 aa, synthetic construct
GGDGVDELE

SEQ ID NO: 32105 - protein, 9 aa, synthetic construct
GGDGVDELH

SEQ ID NO: 32106 - protein, 9 aa, synthetic construct
GGDGVDELQ

SEQ ID NO: 32107 - protein, 9 aa, synthetic construct
GGDGVDEMF

SEQ ID NO: 32108 - protein, 9 aa, synthetic construct
GGDGVDFAS

SEQ ID NO: 32109 - protein, 9 aa, synthetic construct
GGDGVDFIE

SEQ ID NO: 32110 - protein, 9 aa, synthetic construct
GGDGVDFLF

SEQ ID NO: 32111 - protein, 9 aa, synthetic construct
GGDGVDRIY

SEQ ID NO: 32112 - protein, 9 aa, synthetic construct
GGDGVDFLK

SEQ ID NO: 32113 - protein, 9 aa, synthetic construct
GGDGVDFLS

SEQ ID NO: 32114 - protein, 9 aa, synthetic construct
GGDGVDFLT

SEQ ID NO: 32115 - protein, 9 aa, synthetic construct
GGDGVDGAE

SEQ ID NO: 32116 - protein, 9 aa, synthetic construct
GGDGVDGIR

SEQ ID NO: 32117 - protein, 9 aa, synthetic construct
GGDGVDGMA

SEQ ID NO: 32118 - protein, 9 aa, synthetic construct
GGDGVDHIT

SEQ ID NO: 32119 - protein, 9 aa, synthetic construct
GGDGVDHLN

SEQ ID NO: 32120 - protein, 9 aa, synthetic construct
GGDGVDDAY

SEQ ID NO: 32121 - protein, 9 aa, synthetic construct
GGDGVDAYL

SEQ ID NO: 32122 - protein, 9 aa, synthetic construct
GGDGVDAVD

SEQ ID NO: 32123 - protein, 9 aa, synthetic construct
GGDGVDAMT

SEQ ID NO: 32124 - protein, 9 aa, synthetic construct
GGDGTDWLD

SEQ ID NO: 32125 - protein, 9 aa, synthetic construct
GGDGTDWLR

SEQ ID NO: 32126 - protein, 9 aa, synthetic construct
GGDGTDWLS

SEQ ID NO: 32127 - protein, 9 aa, synthetic construct
GGDGTDWLT

SEQ ID NO: 32128 - protein, 9 aa, synthetic construct
GGDGTDYLF

SEQ ID NO: 32129 - protein, 9 aa, synthetic construct
GGDGTDYLL

SEQ ID NO: 32130 - protein, 9 aa, synthetic construct
GGDGTDYLN

SEQ ID NO: 32131 - protein, 9 aa, synthetic construct
GGDGTDYMY

SEQ ID NO: 32132 - protein, 9 aa, synthetic construct
GGDGVDAAS

SEQ ID NO: 32133 - protein, 9 aa, synthetic construct
GGDGVDAFD

SEQ ID NO: 32134 - protein, 9 aa, synthetic construct
GGDGVDAIN

SEQ ID NO: 32135 - protein, 9 aa, synthetic construct
GGDGVDAIQ

SEQ ID NO: 32136 - protein, 9 aa, synthetic construct
GGDGVDALF

SEQ ID NO: 32137 - protein, 9 aa, synthetic construct
GGDGVDALH

SEQ ID NO: 32138 - protein, 9 aa, synthetic construct
GGDGVDALN

SEQ ID NO: 32139 - protein, 9 aa, synthetic construct
GGDGVDALS

SEQ ID NO: 32140 - protein, 9 aa, synthetic construct
GGDGVDALT

SEQ ID NO: 32141 - protein, 9 aa, synthetic construct
GGDGVDHMI

SEQ ID NO: 32142 - protein, 9 aa, synthetic construct
GGDGVDIAD

SEQ ID NO: 32143 - protein, 9 aa, synthetic construct
GGDGVDIAR

SEQ ID NO: 32144 - protein, 9 aa, synthetic construct
GGDGVDLLF

SEQ ID NO: 32145 - protein, 9 aa, synthetic construct
GGDGVDLLY

SEQ ID NO: 32146 - protein, 9 aa, synthetic construct
GGDGVDLVD

SEQ ID NO: 32147 - protein, 9 aa, synthetic construct
GGDGVDMAT

SEQ ID NO: 32148 - protein, 9 aa, synthetic construct
GGDGVDMIL

SEQ ID NO: 32149 - protein, 9 aa, synthetic construct
GGDGVDMIS

SEQ ID NO: 32150 - protein, 9 aa, synthetic construct
GGDGVDMLD

SEQ ID NO: 32151 - protein, 9 aa, synthetic construct
GGDGVDMLS

SEQ ID NO: 32152 - protein, 9 aa, synthetic construct
GGDGVDMLT

SEQ ID NO: 32153 - protein, 9 aa, synthetic construct
GGDGVDNID

SEQ ID NO: 32154 - protein, 9 aa, synthetic construct
GGDGVDNIS

SEQ ID NO: 32155 - protein, 9 aa, synthetic construct
GGDGVDNLL

SEQ ID NO: 32156 - protein, 9 aa, synthetic construct
GGDGVDNLT

SEQ ID NO: 32157 - protein, 9 aa, synthetic construct
GGDGVDQFD

SEQ ID NO: 32158 - protein, 9 aa, synthetic construct
GGDGVDQLE

SEQ ID NO: 32159 - protein, 9 aa, synthetic construct
GGDGVDQLT

SEQ ID NO: 32160 - protein, 9 aa, synthetic construct
GGDGVDQVY

SEQ ID NO: 32161 - protein, 9 aa, synthetic construct
GGDGVDRFT

SEQ ID NO: 32162 - protein, 9 aa, synthetic construct
GGDGVDLLQ

SEQ ID NO: 32163 - protein, 9 aa, synthetic construct
GGDGVDLIS

SEQ ID NO: 32164 - protein, 9 aa, synthetic construct
GGDGVDIAS

SEQ ID NO: 32165 - protein, 9 aa, synthetic construct
GGDGVDLIF

SEQ ID NO: 32166 - protein, 9 aa, synthetic construct
GGDGVDIFK

SEQ ID NO: 32167 - protein, 9 aa, synthetic construct
GGDGVDIIL

SEQ ID NO: 32168 - protein, 9 aa, synthetic construct
GGDGVDIIV

SEQ ID NO: 32169 - protein, 9 aa, synthetic construct
GGDGVDIIY

SEQ ID NO: 32170 - protein, 9 aa, synthetic construct
GGDGVDILD

SEQ ID NO: 32171 - protein, 9 aa, synthetic construct
GGDGVDILF

SEQ ID NO: 32172 - protein, 9 aa, synthetic construct
GGDGVDILY

SEQ ID NO: 32173 - protein, 9 aa, synthetic construct
GGDGVDIMF

SEQ ID NO: 32174 - protein, 9 aa, synthetic construct
GGDGVDIVS

SEQ ID NO: 32175 - protein, 9 aa, synthetic construct
GGDGVDKIV

SEQ ID NO: 32176 - protein, 9 aa, synthetic construct
GGDGVDKIY

SEQ ID NO: 32177 - protein, 9 aa, synthetic construct
GGDGVDKLA

SEQ ID NO: 32178 - protein, 9 aa, synthetic construct
GGDGVDKLN

SEQ ID NO: 32179 - protein, 9 aa, synthetic construct
GGDGVDKLV

SEQ ID NO: 32180 - protein, 9 aa, synthetic construct
GGDGVDLAD

SEQ ID NO: 32181 - protein, 9 aa, synthetic construct
GGDGVDLAN

SEQ ID NO: 32182 - protein, 9 aa, synthetic construct
GGDGVDLFF

SEQ ID NO: 32183 - protein, 9 aa, synthetic construct
GGDGTDWAS

SEQ ID NO: 32184 - protein, 9 aa, synthetic construct
GGDGTDVYW

SEQ ID NO: 32185 - protein, 9 aa, synthetic construct
GGDGTDVVT

SEQ ID NO: 32186 - protein, 9 aa, synthetic construct
GGDGTDLFH

SEQ ID NO: 32187 - protein, 9 aa, synthetic construct
GGDGTDLIL

SEQ ID NO: 32188 - protein, 9 aa, synthetic construct
GGDGTDLIR

SEQ ID NO: 32189 - protein, 9 aa, synthetic construct
GGDGTDLIY

SEQ ID NO: 32190 - protein, 9 aa, synthetic construct
GGDGTDLLH

SEQ ID NO: 32191 - protein, 9 aa, synthetic construct
GGDGTDLLI

SEQ ID NO: 32192 - protein, 9 aa, synthetic construct
GGDGTDLLK

SEQ ID NO: 32193 - protein, 9 aa, synthetic construct
GGDGTDLLS

SEQ ID NO: 32194 - protein, 9 aa, synthetic construct
GGDGTDLMF

SEQ ID NO: 32195 - protein, 9 aa, synthetic construct
GGDGTDLVA

SEQ ID NO: 32196 - protein, 9 aa, synthetic construct
GGDGTDLVD

SEQ ID NO: 32197 - protein, 9 aa, synthetic construct
GGDGTDLVL

SEQ ID NO: 32198 - protein, 9 aa, synthetic construct
GGDGTDLVS

SEQ ID NO: 32199 - protein, 9 aa, synthetic construct
GGDGTDMLL

SEQ ID NO: 32200 - protein, 9 aa, synthetic construct
GGDGTDMLR

SEQ ID NO: 32201 - protein, 9 aa, synthetic construct
GGDGTDMLS

SEQ ID NO: 32202 - protein, 9 aa, synthetic construct
GGDGTDMLY

SEQ ID NO: 32203 - protein, 9 aa, synthetic construct
GGDGTDNAV

SEQ ID NO: 32204 - protein, 9 aa, synthetic construct
GGDGTDLID

SEQ ID NO: 32205 - protein, 9 aa, synthetic construct
GGDGTDLAY

SEQ ID NO: 32206 - protein, 9 aa, synthetic construct
GGDGTDNLY

SEQ ID NO: 32207 - protein, 9 aa, synthetic construct
GGDGTDLAH

SEQ ID NO: 32208 - protein, 9 aa, synthetic construct
GGDGTDHLI

SEQ ID NO: 32209 - protein, 9 aa, synthetic construct
GGDGTDIAM

SEQ ID NO: 32210 - protein, 9 aa, synthetic construct
GGDGTDIAV

SEQ ID NO: 32211 - protein, 9 aa, synthetic construct
GGDGTDIFS

SEQ ID NO: 32212 - protein, 9 aa, synthetic construct
GGDGTDILA

SEQ ID NO: 32213 - protein, 9 aa, synthetic construct
GGDGTDILE

SEQ ID NO: 32214 - protein, 9 aa, synthetic construct
GGDGTDILH

SEQ ID NO: 32215 - protein, 9 aa, synthetic construct
GGDGTDILL

SEQ ID NO: 32216 - protein, 9 aa, synthetic construct
GGDGTDILR

SEQ ID NO: 32217 - protein, 9 aa, synthetic construct
GGDGTDILS

SEQ ID NO: 32218 - protein, 9 aa, synthetic construct
GGDGTDILV

SEQ ID NO: 32219 - protein, 9 aa, synthetic construct
GGDGTDILY

SEQ ID NO: 32220 - protein, 9 aa, synthetic construct
GGDGTDIVL

SEQ ID NO: 32221 - protein, 9 aa, synthetic construct
GGDGTDIVR

SEQ ID NO: 32222 - protein, 9 aa, synthetic construct
GGDGTDKAI

SEQ ID NO: 32223 - protein, 9 aa, synthetic construct
GGDGTDKLL

SEQ ID NO: 32224 - protein, 9 aa, synthetic construct
GGDGTDKLY

SEQ ID NO: 32225 - protein, 9 aa, synthetic construct
GGDGTDNIS

SEQ ID NO: 32226 - protein, 9 aa, synthetic construct
GGDGTDQFN

SEQ ID NO: 32227 - protein, 9 aa, synthetic construct
GGDGTDVVS

SEQ ID NO: 32228 - protein, 9 aa, synthetic construct
GGDGTDTAT

SEQ ID NO: 32229 - protein, 9 aa, synthetic construct
GGDGTDTFI

SEQ ID NO: 32230 - protein, 9 aa, synthetic construct
GGDGTDTFM

SEQ ID NO: 32231 - protein, 9 aa, synthetic construct
GGDGTDTIA

SEQ ID NO: 32232 - protein, 9 aa, synthetic construct
GGDGTDTIV

SEQ ID NO: 32233 - protein, 9 aa, synthetic construct
GGDGTDTLE

SEQ ID NO: 32234 - protein, 9 aa, synthetic construct
GGDGTDTLH

SEQ ID NO: 32235 - protein, 9 aa, synthetic construct
GGDGTDTML

SEQ ID NO: 32236 - protein, 9 aa, synthetic construct
GGDGTDTMT

SEQ ID NO: 32237 - protein, 9 aa, synthetic construct
GGDGTDTVF

SEQ ID NO: 32238 - protein, 9 aa, synthetic construct
GGDGTDTVM

SEQ ID NO: 32239 - protein, 9 aa, synthetic construct
GGDGTDTVN

SEQ ID NO: 32240 - protein, 9 aa, synthetic construct
GGDGTDTYG

SEQ ID NO: 32241 - protein, 9 aa, synthetic construct
GGDGTDTYR

SEQ ID NO: 32242 - protein, 9 aa, synthetic construct
GGDGTDTYV

SEQ ID NO: 32243 - protein, 9 aa, synthetic construct
GGDGTDVLF

SEQ ID NO: 32244 - protein, 9 aa, synthetic construct
GGDGTDVMD

SEQ ID NO: 32245 - protein, 9 aa, synthetic construct
GGDGTDVVQ

SEQ ID NO: 32246 - protein, 9 aa, synthetic construct
GGDGTDTAY

SEQ ID NO: 32247 - protein, 9 aa, synthetic construct
GGDGTDTAN

SEQ ID NO: 32248 - protein, 9 aa, synthetic construct
GGDGTDQID

SEQ ID NO: 32249 - protein, 9 aa, synthetic construct
GGDGTDTAH

SEQ ID NO: 32250 - protein, 9 aa, synthetic construct
GGDGTDQIV

SEQ ID NO: 32251 - protein, 9 aa, synthetic construct
GGDGTDQIW

SEQ ID NO: 32252 - protein, 9 aa, synthetic construct
GGDGTDQLD

SEQ ID NO: 32253 - protein, 9 aa, synthetic construct
GGDGTDQLM

SEQ ID NO: 32254 - protein, 9 aa, synthetic construct
GGDGTDQLR

SEQ ID NO: 32255 - protein, 9 aa, synthetic construct
GGDGTDQLY

SEQ ID NO: 32256 - protein, 9 aa, synthetic construct
GGDGTDRLD

SEQ ID NO: 32257 - protein, 9 aa, synthetic construct
GGDGTDRLF

SEQ ID NO: 32258 - protein, 9 aa, synthetic construct
GGDGTDRVS

SEQ ID NO: 32259 - protein, 9 aa, synthetic construct
GGDGTDRVV

SEQ ID NO: 32260 - protein, 9 aa, synthetic construct
GGDGTDSAS

SEQ ID NO: 32261 - protein, 9 aa, synthetic construct
GGDGTDSFT

SEQ ID NO: 32262 - protein, 9 aa, synthetic construct
GGDGTDSII

SEQ ID NO: 32263 - protein, 9 aa, synthetic construct
GGDGTDSLY

SEQ ID NO: 32264 - protein, 9 aa, synthetic construct
GGDGTDSVD

SEQ ID NO: 32265 - protein, 9 aa, synthetic construct
GGDGTDSVI

SEQ ID NO: 32266 - protein, 9 aa, synthetic construct
GGDGTDTAG

SEQ ID NO: 32267 - protein, 9 aa, synthetic construct
GGDGVDRIF

SEQ ID NO: 32268 - protein, 9 aa, synthetic construct
GGDGVDRLD

SEQ ID NO: 32269 - protein, 9 aa, synthetic construct
GGDGRDDLH

SEQ ID NO: 32270 - protein, 9 aa, synthetic construct
GGDGYDVLV

SEQ ID NO: 32271 - protein, 9 aa, synthetic construct
GGDGYDTYY

SEQ ID NO: 32272 - protein, 9 aa, synthetic construct
GGDGYDVAS

SEQ ID NO: 32273 - protein, 9 aa, synthetic construct
GGDGYDVID

SEQ ID NO: 32274 - protein, 9 aa, synthetic construct
GGDGYDVIN

SEQ ID NO: 32275 - protein, 9 aa, synthetic construct
GGDGYDVIR

SEQ ID NO: 32276 - protein, 9 aa, synthetic construct
GGDGYDVLF

SEQ ID NO: 32277 - protein, 9 aa, synthetic construct
GGDGYDVLL

SEQ ID NO: 32278 - protein, 9 aa, synthetic construct
GGDGYDVLS

SEQ ID NO: 32279 - protein, 9 aa, synthetic construct
GGDGYDWLF

SEQ ID NO: 32280 - protein, 9 aa, synthetic construct
GGDGVDRLE

SEQ ID NO: 32281 - protein, 9 aa, synthetic construct
GGDGYDXLR

SEQ ID NO: 32282 - protein, 9 aa, synthetic construct
GGDGYDYAE

SEQ ID NO: 32283 - protein, 9 aa, synthetic construct
GGDGYDYAL

SEQ ID NO: 32284 - protein, 9 aa, synthetic construct
GGDGYDYFY

SEQ ID NO: 32285 - protein, 9 aa, synthetic construct
GGDGYDYLY

SEQ ID NO: 32286 - protein, 9 aa, synthetic construct
GGEGADAFM

SEQ ID NO: 32287 - protein, 9 aa, synthetic construct
GGEGADAFR

SEQ ID NO: 32288 - protein, 9 aa, synthetic construct
GGEGADAFV

SEQ ID NO: 32289 - protein, 9 aa, synthetic construct
GGDGYDTMG

SEQ ID NO: 32290 - protein, 9 aa, synthetic construct
GGDGYDTMA

SEQ ID NO: 32291 - protein, 9 aa, synthetic construct
GGDGYDTLV

SEQ ID NO: 32292 - protein, 9 aa, synthetic construct
GGDGYDTLT

SEQ ID NO: 32293 - protein, 9 aa, synthetic construct
GGDGYDRFY

SEQ ID NO: 32294 - protein, 9 aa, synthetic construct
GGDGYDRLD

SEQ ID NO: 32295 - protein, 9 aa, synthetic construct
GGDGYDRLF

SEQ ID NO: 32296 - protein, 9 aa, synthetic construct
GGDGYDRLT

SEQ ID NO: 32297 - protein, 9 aa, synthetic construct
GGDGYDSID

SEQ ID NO: 32298 - protein, 9 aa, synthetic construct
GGDGYDSLY

SEQ ID NO: 32299 - protein, 9 aa, synthetic construct
GGDGYDTAA

SEQ ID NO: 32300 - protein, 9 aa, synthetic construct
GGDGYDTAI

SEQ ID NO: 32301 - protein, 9 aa, synthetic construct
GGDGYDTAS

SEQ ID NO: 32302 - protein, 9 aa, synthetic construct
GGDGYDTFV

SEQ ID NO: 32303 - protein, 9 aa, synthetic construct
GGDGYDTIV

SEQ ID NO: 32304 - protein, 9 aa, synthetic construct
GGDGYDTLA

SEQ ID NO: 32305 - protein, 9 aa, synthetic construct
GGDGYDTLE

SEQ ID NO: 32306 - protein, 9 aa, synthetic construct
GGDGYDTLF

SEQ ID NO: 32307 - protein, 9 aa, synthetic construct
GGDGYDTLL

SEQ ID NO: 32308 - protein, 9 aa, synthetic construct
GGDGYDTLN

SEQ ID NO: 32309 - protein, 9 aa, synthetic construct
GGDGYDTLS

SEQ ID NO: 32310 - protein, 9 aa, synthetic construct
GGEGADAIA

SEQ ID NO: 32311 - protein, 9 aa, synthetic construct
GGEGADAIE

SEQ ID NO: 32312 - protein, 9 aa, synthetic construct
GGEGADAIG

SEQ ID NO: 32313 - protein, 9 aa, synthetic construct
GGEGADEIW

SEQ ID NO: 32314 - protein, 9 aa, synthetic construct
GGEGADEMH

SEQ ID NO: 32315 - protein, 9 aa, synthetic construct
GGEGADEMR

SEQ ID NO: 32316 - protein, 9 aa, synthetic construct
GGEGADEMS

SEQ ID NO: 32317 - protein, 9 aa, synthetic construct
GGEGADEMV

SEQ ID NO: 32318 - protein, 9 aa, synthetic construct
GGEGADFAS

SEQ ID NO: 32319 - protein, 9 aa, synthetic construct
GGEGADFIE

SEQ ID NO: 32320 - protein, 9 aa, synthetic construct
GGEGADFIG

SEQ ID NO: 32321 - protein, 9 aa, synthetic construct
GGEGADFLA

SEQ ID NO: 32322 - protein, 9 aa, synthetic construct
GGEGADFLK

SEQ ID NO: 32323 - protein, 9 aa, synthetic construct
GGEGADFLY

SEQ ID NO: 32324 - protein, 9 aa, synthetic construct
GGEGADFMA

SEQ ID NO: 32325 - protein, 9 aa, synthetic construct
GGEGADFVS

SEQ ID NO: 32326 - protein, 9 aa, synthetic construct
GGEGADGFS

SEQ ID NO: 32327 - protein, 9 aa, synthetic construct
GGEGADGIS

SEQ ID NO: 32328 - protein, 9 aa, synthetic construct
GGEGADGLN

SEQ ID NO: 32329 - protein, 9 aa, synthetic construct
GGEGADGLS

SEQ ID NO: 32330 - protein, 9 aa, synthetic construct
GGEGADGVR

SEQ ID NO: 32331 - protein, 9 aa, synthetic construct
GGEGADEMA

SEQ ID NO: 32332 - protein, 9 aa, synthetic construct
GGEGADEIF

SEQ ID NO: 32333 - protein, 9 aa, synthetic construct
GGEGADAIH

SEQ ID NO: 32334 - protein, 9 aa, synthetic construct
GGEGADEID

SEQ ID NO: 32335 - protein, 9 aa, synthetic construct
GGEGADALF

SEQ ID NO: 32336 - protein, 9 aa, synthetic construct
GGEGADALH

SEQ ID NO: 32337 - protein, 9 aa, synthetic construct
GGEGADALL

SEQ ID NO: 32338 - protein, 9 aa, synthetic construct
GGEGADALV

SEQ ID NO: 32339 - protein, 9 aa, synthetic construct
GGEGADALW

SEQ ID NO: 32340 - protein, 9 aa, synthetic construct
GGEGADAMD

SEQ ID NO: 32341 - protein, 9 aa, synthetic construct
GGEGADDFL

SEQ ID NO: 32342 - protein, 9 aa, synthetic construct
GGEGADDFY

SEQ ID NO: 32343 - protein, 9 aa, synthetic construct
GGEGADDII

SEQ ID NO: 32344 - protein, 9 aa, synthetic construct
GGEGADDIY

SEQ ID NO: 32345 - protein, 9 aa, synthetic construct
GGEGADDLD

SEQ ID NO: 32346 - protein, 9 aa, synthetic construct
GGEGADDLH

SEQ ID NO: 32347 - protein, 9 aa, synthetic construct
GGEGADDLI

SEQ ID NO: 32348 - protein, 9 aa, synthetic construct
GGEGADDLL

SEQ ID NO: 32349 - protein, 9 aa, synthetic construct
GGEGADDLS

SEQ ID NO: 32350 - protein, 9 aa, synthetic construct
GGEGADDMY

SEQ ID NO: 32351 - protein, 9 aa, synthetic construct
GGEGADEFY

SEQ ID NO: 32352 - protein, 9 aa, synthetic construct
GGDGYDQMW

SEQ ID NO: 32353 - protein, 9 aa, synthetic construct
GGDGYDQLF

SEQ ID NO: 32354 - protein, 9 aa, synthetic construct
GGDGYDNID

SEQ ID NO: 32355 - protein, 9 aa, synthetic construct
GGDGVDTFT

SEQ ID NO: 32356 - protein, 9 aa, synthetic construct
GGDGVDTIG

SEQ ID NO: 32357 - protein, 9 aa, synthetic construct
GGDGVDTIT

SEQ ID NO: 32358 - protein, 9 aa, synthetic construct
GGDGVDTLE

SEQ ID NO: 32359 - protein, 9 aa, synthetic construct
GGDGVDTLQ

SEQ ID NO: 32360 - protein, 9 aa, synthetic construct
GGDGVDTVI

SEQ ID NO: 32361 - protein, 9 aa, synthetic construct
GGDGVDTVT

SEQ ID NO: 32362 - protein, 9 aa, synthetic construct
GGDGVDTYI

SEQ ID NO: 32363 - protein, 9 aa, synthetic construct
GGDGVDTYL

SEQ ID NO: 32364 - protein, 9 aa, synthetic construct
GGDGVDTYN

SEQ ID NO: 32365 - protein, 9 aa, synthetic construct
GGDGVDTYQ

SEQ ID NO: 32366 - protein, 9 aa, synthetic construct
GGDGVDVLQ

SEQ ID NO: 32367 - protein, 9 aa, synthetic construct
GGDGVDVLT

SEQ ID NO: 32368 - protein, 9 aa, synthetic construct
GGDGVDVLV

SEQ ID NO: 32369 - protein, 9 aa, synthetic construct
GGDGVDVMV

SEQ ID NO: 32370 - protein, 9 aa, synthetic construct
GGDGVDWLV

SEQ ID NO: 32371 - protein, 9 aa, synthetic construct
GGDGVDWVR

SEQ ID NO: 32372 - protein, 9 aa, synthetic construct
GGDGVDYIE

SEQ ID NO: 32373 - protein, 9 aa, synthetic construct
GGDGVDTIE

SEQ ID NO: 32374 - protein, 9 aa, synthetic construct
GGDGVDTAM

SEQ ID NO: 32375 - protein, 9 aa, synthetic construct
GGDGWDAVY

SEQ ID NO: 32376 - protein, 9 aa, synthetic construct
GGDGVDTAG

SEQ ID NO: 32377 - protein, 9 aa, synthetic construct
GGDGVDRLF

SEQ ID NO: 32378 - protein, 9 aa, synthetic construct
GGDGVDRLI

SEQ ID NO: 32379 - protein, 9 aa, synthetic construct
GGDGVDRLK

SEQ ID NO: 32380 - protein, 9 aa, synthetic construct
GGDGVDRLL

SEQ ID NO: 32381 - protein, 9 aa, synthetic construct
GGDGVDRLR

SEQ ID NO: 32382 - protein, 9 aa, synthetic construct
GGDGVDRLW

SEQ ID NO: 32383 - protein, 9 aa, synthetic construct
GGDGVDRVW

SEQ ID NO: 32384 - protein, 9 aa, synthetic construct
GGDGVDSLD

SEQ ID NO: 32385 - protein, 9 aa, synthetic construct
GGDGVDSLE

SEQ ID NO: 32386 - protein, 9 aa, synthetic construct
GGDGVDSLN

SEQ ID NO: 32387 - protein, 9 aa, synthetic construct
GGDGVDSLQ

SEQ ID NO: 32388 - protein, 9 aa, synthetic construct
GGDGVDSLS

SEQ ID NO: 32389 - protein, 9 aa, synthetic construct
GGDGVDSLV

SEQ ID NO: 32390 - protein, 9 aa, synthetic construct
GGDGVDSMA

SEQ ID NO: 32391 - protein, 9 aa, synthetic construct
GGDGVDSMN

SEQ ID NO: 32392 - protein, 9 aa, synthetic construct
GGDGVDTAA

SEQ ID NO: 32393 - protein, 9 aa, synthetic construct
GGDGVDTAE

SEQ ID NO: 32394 - protein, 9 aa, synthetic construct
GGDGVDYVA

SEQ ID NO: 32395 - protein, 9 aa, synthetic construct
GGDGWDDLR

SEQ ID NO: 32396 - protein, 9 aa, synthetic construct
GGDGYDLLY

SEQ ID NO: 32397 - protein, 9 aa, synthetic construct
GGDGXDSID

SEQ ID NO: 32398 - protein, 9 aa, synthetic construct
GGDGYDAFY

SEQ ID NO: 32399 - protein, 9 aa, synthetic construct
GGDGYDALF

SEQ ID NO: 32400 - protein, 9 aa, synthetic construct
GGDGYDALQ

SEQ ID NO: 32401 - protein, 9 aa, synthetic construct
GGDGYDALS

SEQ ID NO: 32402 - protein, 9 aa, synthetic construct
GGDGYDDLL

SEQ ID NO: 32403 - protein, 9 aa, synthetic construct
GGDGYDDVY

SEQ ID NO: 32404 - protein, 9 aa, synthetic construct
GGDGYDHLY

SEQ ID NO: 32405 - protein, 9 aa, synthetic construct
GGDGYDHYW

SEQ ID NO: 32406 - protein, 9 aa, synthetic construct
GGDGYDILI

SEQ ID NO: 32407 - protein, 9 aa, synthetic construct
GGDGYDILY

SEQ ID NO: 32408 - protein, 9 aa, synthetic construct
GGDGYDIVS

SEQ ID NO: 32409 - protein, 9 aa, synthetic construct
GGDGYDKIQ

SEQ ID NO: 32410 - protein, 9 aa, synthetic construct
GGDGYDKLS

SEQ ID NO: 32411 - protein, 9 aa, synthetic construct
GGDGYDLFL

SEQ ID NO: 32412 - protein, 9 aa, synthetic construct
GGDGYDLIA

SEQ ID NO: 32413 - protein, 9 aa, synthetic construct
GGDGYDLIW

SEQ ID NO: 32414 - protein, 9 aa, synthetic construct
GGDGYDLLE

SEQ ID NO: 32415 - protein, 9 aa, synthetic construct
GGDGXDSLV

SEQ ID NO: 32416 - protein, 9 aa, synthetic construct
GGDGWDVVS

SEQ ID NO: 32417 - protein, 9 aa, synthetic construct
GGDGWDFLV

SEQ ID NO: 32418 - protein, 9 aa, synthetic construct
GGDGWDVVR

SEQ ID NO: 32419 - protein, 9 aa, synthetic construct
GGDGWDILC

SEQ ID NO: 32420 - protein, 9 aa, synthetic construct
GGDGWDLIA

SEQ ID NO: 32421 - protein, 9 aa, synthetic construct
GGDGWDLLD

SEQ ID NO: 32422 - protein, 9 aa, synthetic construct
GGDGWDLLE

SEQ ID NO: 32423 - protein, 9 aa, synthetic construct
GGDGWDLMF

SEQ ID NO: 32424 - protein, 9 aa, synthetic construct
GGDGWDMAV

SEQ ID NO: 32425 - protein, 9 aa, synthetic construct
GGDGWDNLN

SEQ ID NO: 32426 - protein, 9 aa, synthetic construct
GGDGWDNVR

SEQ ID NO: 32427 - protein, 9 aa, synthetic construct
GGDGWDQVN

SEQ ID NO: 32428 - protein, 9 aa, synthetic construct
GGDGWDSLV

SEQ ID NO: 32429 - protein, 9 aa, synthetic construct
GGDGWDTIF

SEQ ID NO: 32430 - protein, 9 aa, synthetic construct
GGDGWDTIH

SEQ ID NO: 32431 - protein, 9 aa, synthetic construct
GGDGWDTLI

SEQ ID NO: 32432 - protein, 9 aa, synthetic construct
GGDGWDTVR

SEQ ID NO: 32433 - protein, 9 aa, synthetic construct
GGDGWDTVS

SEQ ID NO: 32434 - protein, 9 aa, synthetic construct
GGDGWDVIF

SEQ ID NO: 32435 - protein, 9 aa, synthetic construct
GGDGWDVLY

SEQ ID NO: 32436 - protein, 9 aa, synthetic construct
GGDGTDHLA

SEQ ID NO: 32437 - protein, 9 aa, synthetic construct
GGDGTDHIY

SEQ ID NO: 32438 - protein, 9 aa, synthetic construct
GGDGTDHIH

SEQ ID NO: 32439 - protein, 9 aa, synthetic construct
GGDGRDTVF

SEQ ID NO: 32440 - protein, 9 aa, synthetic construct
GGDGRDTLK

SEQ ID NO: 32441 - protein, 9 aa, synthetic construct
GGDGRDTLQ

SEQ ID NO: 32442 - protein, 9 aa, synthetic construct
GGDGRDTLY

SEQ ID NO: 32443 - protein, 9 aa, synthetic construct
GGDGRDTMD

SEQ ID NO: 32444 - protein, 9 aa, synthetic construct
GGDGRDTML

SEQ ID NO: 32445 - protein, 9 aa, synthetic construct
GGDGRDTMQ

SEQ ID NO: 32446 - protein, 9 aa, synthetic construct
GGDGRDTMT

SEQ ID NO: 32447 - protein, 9 aa, synthetic construct
GGDGRDTMY

SEQ ID NO: 32448 - protein, 9 aa, synthetic construct
GGDGRDTVI

SEQ ID NO: 32449 - protein, 9 aa, synthetic construct
GGDGTDFMV

SEQ ID NO: 32450 - protein, 9 aa, synthetic construct
GGDGRDTVM

SEQ ID NO: 32451 - protein, 9 aa, synthetic construct
GGDGRDVAE

SEQ ID NO: 32452 - protein, 9 aa, synthetic construct
GGDGRDVIN

SEQ ID NO: 32453 - protein, 9 aa, synthetic construct
GGDGRDVIR

SEQ ID NO: 32454 - protein, 9 aa, synthetic construct
GGDGRDVLA

SEQ ID NO: 32455 - protein, 9 aa, synthetic construct
GGDGRDVLE

SEQ ID NO: 32456 - protein, 9 aa, synthetic construct
GGDGRDVMD

SEQ ID NO: 32457 - protein, 9 aa, synthetic construct
GGDGRDVMR

SEQ ID NO: 32458 - protein, 9 aa, synthetic construct
GGDGRDTLH

SEQ ID NO: 32459 - protein, 9 aa, synthetic construct
GGDGRDTIT

SEQ ID NO: 32460 - protein, 9 aa, synthetic construct
GGDGRDTIL

SEQ ID NO: 32461 - protein, 9 aa, synthetic construct
GGDGRDTIE

SEQ ID NO: 32462 - protein, 9 aa, synthetic construct
GGDGRDSIA

SEQ ID NO: 32463 - protein, 9 aa, synthetic construct
GGDGRDSID

SEQ ID NO: 32464 - protein, 9 aa, synthetic construct
GGDGRDSIE

SEQ ID NO: 32465 - protein, 9 aa, synthetic construct
GGDGRDSIR

SEQ ID NO: 32466 - protein, 9 aa, synthetic construct
GGDGRDSIS

SEQ ID NO: 32467 - protein, 9 aa, synthetic construct
GGDGRDSLI

SEQ ID NO: 32468 - protein, 9 aa, synthetic construct
GGDGRDSLN

SEQ ID NO: 32469 - protein, 9 aa, synthetic construct
GGDGRDSLQ

SEQ ID NO: 32470 - protein, 9 aa, synthetic construct
GGDGRDSLR

SEQ ID NO: 32471 - protein, 9 aa, synthetic construct
GGDGRDSVN

SEQ ID NO: 32472 - protein, 9 aa, synthetic construct
GGDGRDTAA

SEQ ID NO: 32473 - protein, 9 aa, synthetic construct
GGDGRDTAD

SEQ ID NO: 32474 - protein, 9 aa, synthetic construct
GGDGRDTAL

SEQ ID NO: 32475 - protein, 9 aa, synthetic construct
GGDGRDTAV

SEQ ID NO: 32476 - protein, 9 aa, synthetic construct
GGDGRDTAY

SEQ ID NO: 32477 - protein, 9 aa, synthetic construct
GGDGRDTFM

SEQ ID NO: 32478 - protein, 9 aa, synthetic construct
GGDGRDTFR

SEQ ID NO: 32479 - protein, 9 aa, synthetic construct
GGDGRDVMY

SEQ ID NO: 32480 - protein, 9 aa, synthetic construct
GGDGRDVVI

SEQ ID NO: 32481 - protein, 9 aa, synthetic construct
GGDGRDVVW

SEQ ID NO: 32482 - protein, 9 aa, synthetic construct
GGDGSDDLI

SEQ ID NO: 32483 - protein, 9 aa, synthetic construct
GGDGSDDLQ

SEQ ID NO: 32484 - protein, 9 aa, synthetic construct
GGDGSDDLS

SEQ ID NO: 32485 - protein, 9 aa, synthetic construct
GGDGSDDMG

SEQ ID NO: 32486 - protein, 9 aa, synthetic construct
GGDGSDDVW

SEQ ID NO: 32487 - protein, 9 aa, synthetic construct
GGDGSDEIF

SEQ ID NO: 32488 - protein, 9 aa, synthetic construct
GGDGSDEIH

SEQ ID NO: 32489 - protein, 9 aa, synthetic construct
GGDGSDEIN

SEQ ID NO: 32490 - protein, 9 aa, synthetic construct
GGDGSDEIR

SEQ ID NO: 32491 - protein, 9 aa, synthetic construct
GGDGSDEIV

SEQ ID NO: 32492 - protein, 9 aa, synthetic construct
GGDGSDELH

SEQ ID NO: 32493 - protein, 9 aa, synthetic construct
GGDGSDELL

SEQ ID NO: 32494 - protein, 9 aa, synthetic construct
GGDGSDELN

SEQ ID NO: 32495 - protein, 9 aa, synthetic construct
GGDGSDELT

SEQ ID NO: 32496 - protein, 9 aa, synthetic construct
GGDGSDELV

SEQ ID NO: 32497 - protein, 9 aa, synthetic construct
GGDGSDEMT

SEQ ID NO: 32498 - protein, 9 aa, synthetic construct
GGDGSDEVH

SEQ ID NO: 32499 - protein, 9 aa, synthetic construct
GGDGSDFIM

SEQ ID NO: 32500 - protein, 9 aa, synthetic construct
GGDGSDDLN

SEQ ID NO: 32501 - protein, 9 aa, synthetic construct
GGDGSDDLF

SEQ ID NO: 32502 - protein, 9 aa, synthetic construct
GGDGRDWAD

SEQ ID NO: 32503 - protein, 9 aa, synthetic construct
GGDGSDDFF

SEQ ID NO: 32504 - protein, 9 aa, synthetic construct
GGDGRDWID

SEQ ID NO: 32505 - protein, 9 aa, synthetic construct
GGDGRDWLA

SEQ ID NO: 32506 - protein, 9 aa, synthetic construct
GGDGRDWLE

SEQ ID NO: 32507 - protein, 9 aa, synthetic construct
GGDGRDWLF

SEQ ID NO: 32508 - protein, 9 aa, synthetic construct
GGDGRDWLH

SEQ ID NO: 32509 - protein, 9 aa, synthetic construct
GGDGRDWLI

SEQ ID NO: 32510 - protein, 9 aa, synthetic construct
GGDGRDWLT

SEQ ID NO: 32511 - protein, 9 aa, synthetic construct
GGDGRDYFV

SEQ ID NO: 32512 - protein, 9 aa, synthetic construct
GGDGRDYLN

SEQ ID NO: 32513 - protein, 9 aa, synthetic construct
GGDGRDYLS

SEQ ID NO: 32514 - protein, 9 aa, synthetic construct
GGDGRDYLW

SEQ ID NO: 32515 - protein, 9 aa, synthetic construct
GGDGRDYVA

SEQ ID NO: 32516 - protein, 9 aa, synthetic construct
GGDGRDYVQ

SEQ ID NO: 32517 - protein, 9 aa, synthetic construct
GGDGSDALI

SEQ ID NO: 32518 - protein, 9 aa, synthetic construct
GGDGSDALS

SEQ ID NO: 32519 - protein, 9 aa, synthetic construct
GGDGSDAVA

SEQ ID NO: 32520 - protein, 9 aa, synthetic construct
GGDGSDAYF

SEQ ID NO: 32521 - protein, 9 aa, synthetic construct
GGDGRDSFV

SEQ ID NO: 32522 - protein, 9 aa, synthetic construct
GGDGRDSFQ

SEQ ID NO: 32523 - protein, 9 aa, synthetic construct
GGDGRDSAS

SEQ ID NO: 32524 - protein, 9 aa, synthetic construct
GGDGRDIIF

SEQ ID NO: 32525 - protein, 9 aa, synthetic construct
GGDGRDILE

SEQ ID NO: 32526 - protein, 9 aa, synthetic construct
GGDGRDILM

SEQ ID NO: 32527 - protein, 9 aa, synthetic construct
GGDGRDILY

SEQ ID NO: 32528 - protein, 9 aa, synthetic construct
GGDGRDKID

SEQ ID NO: 32529 - protein, 9 aa, synthetic construct
GGDGRDKIE

SEQ ID NO: 32530 - protein, 9 aa, synthetic construct
GGDGRDKII

SEQ ID NO: 32531 - protein, 9 aa, synthetic construct
GGDGRDKIK

SEQ ID NO: 32532 - protein, 9 aa, synthetic construct
GGDGRDKIS

SEQ ID NO: 32533 - protein, 9 aa, synthetic construct
GGDGRDKLK

SEQ ID NO: 32534 - protein, 9 aa, synthetic construct
GGDGRDKLN

SEQ ID NO: 32535 - protein, 9 aa, synthetic construct
GGDGRDKLT

SEQ ID NO: 32536 - protein, 9 aa, synthetic construct
GGDGRDKLW

SEQ ID NO: 32537 - protein, 9 aa, synthetic construct
GGDGRDKVY

SEQ ID NO: 32538 - protein, 9 aa, synthetic construct
GGDGRDLAD

SEQ ID NO: 32539 - protein, 9 aa, synthetic construct
GGDGRDLFI

SEQ ID NO: 32540 - protein, 9 aa, synthetic construct
GGDGRDLIA

SEQ ID NO: 32541 - protein, 9 aa, synthetic construct
GGDGRDLIF

SEQ ID NO: 32542 - protein, 9 aa, synthetic construct
GGDGRDIIV

SEQ ID NO: 32543 - protein, 9 aa, synthetic construct
GGDGRDIIE

SEQ ID NO: 32544 - protein, 9 aa, synthetic construct
GGDGRDLIT

SEQ ID NO: 32545 - protein, 9 aa, synthetic construct
GGDGRDHLY

SEQ ID NO: 32546 - protein, 9 aa, synthetic construct
GGDGRDDLK

SEQ ID NO: 32547 - protein, 9 aa, synthetic construct
GGDGRDDLR

SEQ ID NO: 32548 - protein, 9 aa, synthetic construct
GGDGRDDLT

SEQ ID NO: 32549 - protein, 9 aa, synthetic construct
GGDGRDDMW

SEQ ID NO: 32550 - protein, 9 aa, synthetic construct
GGDGRDELD

SEQ ID NO: 32551 - protein, 9 aa, synthetic construct
GGDGRDELI

SEQ ID NO: 32552 - protein, 9 aa, synthetic construct
GGDGRDELL

SEQ ID NO: 32553 - protein, 9 aa, synthetic construct
GGDGRDFID

SEQ ID NO: 32554 - protein, 9 aa, synthetic construct
GGDGRDFLD

SEQ ID NO: 32555 - protein, 9 aa, synthetic construct
GGDGRDFLF

SEQ ID NO: 32556 - protein, 9 aa, synthetic construct
GGDGRDFLR

SEQ ID NO: 32557 - protein, 9 aa, synthetic construct
GGDGRDFLS

SEQ ID NO: 32558 - protein, 9 aa, synthetic construct
GGDGRDFLV

SEQ ID NO: 32559 - protein, 9 aa, synthetic construct
GGDGRDHAD

SEQ ID NO: 32560 - protein, 9 aa, synthetic construct
GGDGRDHLI

SEQ ID NO: 32561 - protein, 9 aa, synthetic construct
GGDGRDHLL

SEQ ID NO: 32562 - protein, 9 aa, synthetic construct
GGDGRDHLR

SEQ ID NO: 32563 - protein, 9 aa, synthetic construct
GGDGRDLIH

SEQ ID NO: 32564 - protein, 9 aa, synthetic construct
GGDGRDLIV

SEQ ID NO: 32565 - protein, 9 aa, synthetic construct
GGDGRDRVT

SEQ ID NO: 32566 - protein, 9 aa, synthetic construct
GGDGRDNLR

SEQ ID NO: 32567 - protein, 9 aa, synthetic construct
GGDGRDQIN

SEQ ID NO: 32568 - protein, 9 aa, synthetic construct
GGDGRDQIS

SEQ ID NO: 32569 - protein, 9 aa, synthetic construct
GGDGRDQIY

SEQ ID NO: 32570 - protein, 9 aa, synthetic construct
GGDGRDQLI

SEQ ID NO: 32571 - protein, 9 aa, synthetic construct
GGDGRDQLR

SEQ ID NO: 32572 - protein, 9 aa, synthetic construct
GGDGRDQLW

SEQ ID NO: 32573 - protein, 9 aa, synthetic construct
GGDGRDQLY

SEQ ID NO: 32574 - protein, 9 aa, synthetic construct
GGDGRDRFD

SEQ ID NO: 32575 - protein, 9 aa, synthetic construct
GGDGRDRFE

SEQ ID NO: 32576 - protein, 9 aa, synthetic construct
GGDGRDRIF

SEQ ID NO: 32577 - protein, 9 aa, synthetic construct
GGDGRDRIG

SEQ ID NO: 32578 - protein, 9 aa, synthetic construct
GGDGRDRIK

SEQ ID NO: 32579 - protein, 9 aa, synthetic construct
GGDGRDRIQ

SEQ ID NO: 32580 - protein, 9 aa, synthetic construct
GGDGRDRLC

SEQ ID NO: 32581 - protein, 9 aa, synthetic construct
GGDGRDRLN

SEQ ID NO: 32582 - protein, 9 aa, synthetic construct
GGDGRDRMD

SEQ ID NO: 32583 - protein, 9 aa, synthetic construct
GGDGRDRVA

SEQ ID NO: 32584 - protein, 9 aa, synthetic construct
GGDGRDNLS

SEQ ID NO: 32585 - protein, 9 aa, synthetic construct
GGDGRDNLN

SEQ ID NO: 32586 - protein, 9 aa, synthetic construct
GGDGRDLLA

SEQ ID NO: 32587 - protein, 9 aa, synthetic construct
GGDGRDNLI

SEQ ID NO: 32588 - protein, 9 aa, synthetic construct
GGDGRDLLR

SEQ ID NO: 32589 - protein, 9 aa, synthetic construct
GGDGRDLLS

SEQ ID NO: 32590 - protein, 9 aa, synthetic construct
GGDGRDLVD

SEQ ID NO: 32591 - protein, 9 aa, synthetic construct
GGDGRDLVL

SEQ ID NO: 32592 - protein, 9 aa, synthetic construct
GGDGRDLVQ

SEQ ID NO: 32593 - protein, 9 aa, synthetic construct
GGDGRDLVS

SEQ ID NO: 32594 - protein, 9 aa, synthetic construct
GGDGRDLVT

SEQ ID NO: 32595 - protein, 9 aa, synthetic construct
GGDGRDLVW

SEQ ID NO: 32596 - protein, 9 aa, synthetic construct
GGDGRDMLA

SEQ ID NO: 32597 - protein, 9 aa, synthetic construct
GGDGRDMLG

SEQ ID NO: 32598 - protein, 9 aa, synthetic construct
GGDGRDMLS

SEQ ID NO: 32599 - protein, 9 aa, synthetic construct
GGDGRDMLV

SEQ ID NO: 32600 - protein, 9 aa, synthetic construct
GGDGRDNIN

SEQ ID NO: 32601 - protein, 9 aa, synthetic construct
GGDGRDNIS

SEQ ID NO: 32602 - protein, 9 aa, synthetic construct
GGDGRDNLD

SEQ ID NO: 32603 - protein, 9 aa, synthetic construct
GGDGRDNLG

SEQ ID NO: 32604 - protein, 9 aa, synthetic construct
GGDGRDNLH

SEQ ID NO: 32605 - protein, 9 aa, synthetic construct
GGDGSDFIN

SEQ ID NO: 32606 - protein, 9 aa, synthetic construct
GGDGSDFIS

SEQ ID NO: 32607 - protein, 9 aa, synthetic construct
GGDGSDFLD

SEQ ID NO: 32608 - protein, 9 aa, synthetic construct
GGDGSDTIR

SEQ ID NO: 32609 - protein, 9 aa, synthetic construct
GGDGSDTMD

SEQ ID NO: 32610 - protein, 9 aa, synthetic construct
GGDGSDTMN

SEQ ID NO: 32611 - protein, 9 aa, synthetic construct
GGDGSDTVA

SEQ ID NO: 32612 - protein, 9 aa, synthetic construct
GGDGSDTVE

SEQ ID NO: 32613 - protein, 9 aa, synthetic construct
GGDGSDTVF

SEQ ID NO: 32614 - protein, 9 aa, synthetic construct
GGDGSDTVH

SEQ ID NO: 32615 - protein, 9 aa, synthetic construct
GGDGSDTVI

SEQ ID NO: 32616 - protein, 9 aa, synthetic construct
GGDGSDTVS

SEQ ID NO: 32617 - protein, 9 aa, synthetic construct
GGDGSDTYA

SEQ ID NO: 32618 - protein, 9 aa, synthetic construct
GGDGSDTYD

SEQ ID NO: 32619 - protein, 9 aa, synthetic construct
GGDGSDTYE

SEQ ID NO: 32620 - protein, 9 aa, synthetic construct
GGDGSDTYH

SEQ ID NO: 32621 - protein, 9 aa, synthetic construct
GGDGSDTYT

SEQ ID NO: 32622 - protein, 9 aa, synthetic construct
GGDGSDVFA

SEQ ID NO: 32623 - protein, 9 aa, synthetic construct
GGDGSDVFF

SEQ ID NO: 32624 - protein, 9 aa, synthetic construct
GGDGSDVFM

SEQ ID NO: 32625 - protein, 9 aa, synthetic construct
GGDGSDVIQ

SEQ ID NO: 32626 - protein, 9 aa, synthetic construct
GGDGSDTLM

SEQ ID NO: 32627 - protein, 9 aa, synthetic construct
GGDGSDTIQ

SEQ ID NO: 32628 - protein, 9 aa, synthetic construct
GGDGSDVLK

SEQ ID NO: 32629 - protein, 9 aa, synthetic construct
GGDGSDTFN

SEQ ID NO: 32630 - protein, 9 aa, synthetic construct
GGDGSDRVT

SEQ ID NO: 32631 - protein, 9 aa, synthetic construct
GGDGSDRVY

SEQ ID NO: 32632 - protein, 9 aa, synthetic construct
GGDGSDRYY

SEQ ID NO: 32633 - protein, 9 aa, synthetic construct
GGDGSDSAF

SEQ ID NO: 32634 - protein, 9 aa, synthetic construct
GGDGSDSAS

SEQ ID NO: 32635 - protein, 9 aa, synthetic construct
GGDGSDSIQ

SEQ ID NO: 32636 - protein, 9 aa, synthetic construct
GGDGSDSIT

SEQ ID NO: 32637 - protein, 9 aa, synthetic construct
GGDGSDSLC

SEQ ID NO: 32638 - protein, 9 aa, synthetic construct
GGDGSDSLE

SEQ ID NO: 32639 - protein, 9 aa, synthetic construct
GGDGSDSLH

SEQ ID NO: 32640 - protein, 9 aa, synthetic construct
GGDGSDSLN

SEQ ID NO: 32641 - protein, 9 aa, synthetic construct
GGDGSDSLQ

SEQ ID NO: 32642 - protein, 9 aa, synthetic construct
GGDGSDSVI

SEQ ID NO: 32643 - protein, 9 aa, synthetic construct
GGDGSDSVT

SEQ ID NO: 32644 - protein, 9 aa, synthetic construct
GGDGSDTAA

SEQ ID NO: 32645 - protein, 9 aa, synthetic construct
GGDGSDTAG

SEQ ID NO: 32646 - protein, 9 aa, synthetic construct
GGDGSDTFI

SEQ ID NO: 32647 - protein, 9 aa, synthetic construct
GGDGSDVIR

SEQ ID NO: 32648 - protein, 9 aa, synthetic construct
GGDGSDVMK

SEQ ID NO: 32649 - protein, 9 aa, synthetic construct
GGDGSDRMN

SEQ ID NO: 32650 - protein, 9 aa, synthetic construct
GGDGSDYVY

SEQ ID NO: 32651 - protein, 9 aa, synthetic construct
GGDGTDAAD

SEQ ID NO: 32652 - protein, 9 aa, synthetic construct
GGDGTDAAH

SEQ ID NO: 32653 - protein, 9 aa, synthetic construct
GGDGTDAAL

SEQ ID NO: 32654 - protein, 9 aa, synthetic construct
GGDGTDAIL

SEQ ID NO: 32655 - protein, 9 aa, synthetic construct
GGDGTDALA

SEQ ID NO: 32656 - protein, 9 aa, synthetic construct
GGDGTDAVY

SEQ ID NO: 32657 - protein, 9 aa, synthetic construct
GGDGTDDIS

SEQ ID NO: 32658 - protein, 9 aa, synthetic construct
GGDGTDDLG

SEQ ID NO: 32659 - protein, 9 aa, synthetic construct
GGDGTDEIG

SEQ ID NO: 32660 - protein, 9 aa, synthetic construct
GGDGTDEIN

SEQ ID NO: 32661 - protein, 9 aa, synthetic construct
GGDGTDELE

SEQ ID NO: 32662 - protein, 9 aa, synthetic construct
GGDGTDELQ

SEQ ID NO: 32663 - protein, 9 aa, synthetic construct
GGDGTDFIN

SEQ ID NO: 32664 - protein, 9 aa, synthetic construct
GGDGTDFIS

SEQ ID NO: 32665 - protein, 9 aa, synthetic construct
GGDGTDFLH

SEQ ID NO: 32666 - protein, 9 aa, synthetic construct
GGDGTDFLR

SEQ ID NO: 32667 - protein, 9 aa, synthetic construct
GGDGTDFLY

SEQ ID NO: 32668 - protein, 9 aa, synthetic construct
GGDGSDYYI

SEQ ID NO: 32669 - protein, 9 aa, synthetic construct
GGDGSDYVE

SEQ ID NO: 32670 - protein, 9 aa, synthetic construct
GGDGSDVMY

SEQ ID NO: 32671 - protein, 9 aa, synthetic construct
GGDGSDYMS

SEQ ID NO: 32672 - protein, 9 aa, synthetic construct
GGDGSDVVA

SEQ ID NO: 32673 - protein, 9 aa, synthetic construct
GGDGSDVVQ

SEQ ID NO: 32674 - protein, 9 aa, synthetic construct
GGDGSDVVS

SEQ ID NO: 32675 - protein, 9 aa, synthetic construct
GGDGSDVYF

SEQ ID NO: 32676 - protein, 9 aa, synthetic construct
GGDGSDVYK

SEQ ID NO: 32677 - protein, 9 aa, synthetic construct
GGDGSDVYY

SEQ ID NO: 32678 - protein, 9 aa, synthetic construct
GGDGSDWLE

SEQ ID NO: 32679 - protein, 9 aa, synthetic construct
GGDGSDWLL

SEQ ID NO: 32680 - protein, 9 aa, synthetic construct
GGDGSDWLN

SEQ ID NO: 32681 - protein, 9 aa, synthetic construct
GGDGSDWLW

SEQ ID NO: 32682 - protein, 9 aa, synthetic construct
GGDGSDWLY

SEQ ID NO: 32683 - protein, 9 aa, synthetic construct
GGDGSDWME

SEQ ID NO: 32684 - protein, 9 aa, synthetic construct
GGDGSDWVS

SEQ ID NO: 32685 - protein, 9 aa, synthetic construct
GGDGSDWVW

SEQ ID NO: 32686 - protein, 9 aa, synthetic construct
GGDGSDYLM

SEQ ID NO: 32687 - protein, 9 aa, synthetic construct
GGDGSDYLQ

SEQ ID NO: 32688 - protein, 9 aa, synthetic construct
GGDGSDYLV

SEQ ID NO: 32689 - protein, 9 aa, synthetic construct
GGDGSDRMV

SEQ ID NO: 32690 - protein, 9 aa, synthetic construct
GGDGSDRME

SEQ ID NO: 32691 - protein, 9 aa, synthetic construct
GGDGSDFLF

SEQ ID NO: 32692 - protein, 9 aa, synthetic construct
GGDGSDIFS

SEQ ID NO: 32693 - protein, 9 aa, synthetic construct
GGDGSDIIN

SEQ ID NO: 32694 - protein, 9 aa, synthetic construct
GGDGSDIIT

SEQ ID NO: 32695 - protein, 9 aa, synthetic construct
GGDGSDILG

SEQ ID NO: 32696 - protein, 9 aa, synthetic construct
GGDGSDILK

SEQ ID NO: 32697 - protein, 9 aa, synthetic construct
GGDGSDILL

SEQ ID NO: 32698 - protein, 9 aa, synthetic construct
GGDGSDILR

SEQ ID NO: 32699 - protein, 9 aa, synthetic construct
GGDGSDILS

SEQ ID NO: 32700 - protein, 9 aa, synthetic construct
GGDGSDIYQ

SEQ ID NO: 32701 - protein, 9 aa, synthetic construct
GGDGSDIYR

SEQ ID NO: 32702 - protein, 9 aa, synthetic construct
GGDGSDIYS

SEQ ID NO: 32703 - protein, 9 aa, synthetic construct
GGDGSDKIK

SEQ ID NO: 32704 - protein, 9 aa, synthetic construct
GGDGSDKIL

SEQ ID NO: 32705 - protein, 9 aa, synthetic construct
GGDGSDKLH

SEQ ID NO: 32706 - protein, 9 aa, synthetic construct
GGDGSDKLI

SEQ ID NO: 32707 - protein, 9 aa, synthetic construct
GGDGSDKLT

SEQ ID NO: 32708 - protein, 9 aa, synthetic construct
GGDGSDKLW

SEQ ID NO: 32709 - protein, 9 aa, synthetic construct
GGDGSDKML

SEQ ID NO: 32710 - protein, 9 aa, synthetic construct
GGDGSDIII

SEQ ID NO: 32711 - protein, 9 aa, synthetic construct
GGDGSDIFR

SEQ ID NO: 32712 - protein, 9 aa, synthetic construct
GGDGSDLFV

SEQ ID NO: 32713 - protein, 9 aa, synthetic construct
GGDGSDIAS

SEQ ID NO: 32714 - protein, 9 aa, synthetic construct
GGDGSDFLG

SEQ ID NO: 32715 - protein, 9 aa, synthetic construct
GGDGSDFLI

SEQ ID NO: 32716 - protein, 9 aa, synthetic construct
GGDGSDFLQ

SEQ ID NO: 32717 - protein, 9 aa, synthetic construct
GGDGSDFLS

SEQ ID NO: 32718 - protein, 9 aa, synthetic construct
GGDGSDFLV

SEQ ID NO: 32719 - protein, 9 aa, synthetic construct
GGDGSDFMM

SEQ ID NO: 32720 - protein, 9 aa, synthetic construct
GGDGSDFMT

SEQ ID NO: 32721 - protein, 9 aa, synthetic construct
GGDGSDFVR

SEQ ID NO: 32722 - protein, 9 aa, synthetic construct
GGDGSDFVS

SEQ ID NO: 32723 - protein, 9 aa, synthetic construct
GGDGSDFYL

SEQ ID NO: 32724 - protein, 9 aa, synthetic construct
GGDGSDGIY

SEQ ID NO: 32725 - protein, 9 aa, synthetic construct
GGDGSDGLF

SEQ ID NO: 32726 - protein, 9 aa, synthetic construct
GGDGSDHIF

SEQ ID NO: 32727 - protein, 9 aa, synthetic construct
GGDGSDHIY

SEQ ID NO: 32728 - protein, 9 aa, synthetic construct
GGDGSDHLR

SEQ ID NO: 32729 - protein, 9 aa, synthetic construct
GGDGSDHLT

SEQ ID NO: 32730 - protein, 9 aa, synthetic construct
GGDGSDIAN

SEQ ID NO: 32731 - protein, 9 aa, synthetic construct
GGDGSDLFI

SEQ ID NO: 32732 - protein, 9 aa, synthetic construct
GGDGSDLIL

SEQ ID NO: 32733 - protein, 9 aa, synthetic construct
GGDGSDRMD

SEQ ID NO: 32734 - protein, 9 aa, synthetic construct
GGDGSDQFK

SEQ ID NO: 32735 - protein, 9 aa, synthetic construct
GGDGSDQID

SEQ ID NO: 32736 - protein, 9 aa, synthetic construct
GGDGSDQIY

SEQ ID NO: 32737 - protein, 9 aa, synthetic construct
GGDGSDQLA

SEQ ID NO: 32738 - protein, 9 aa, synthetic construct
GGDGSDQLH

SEQ ID NO: 32739 - protein, 9 aa, synthetic construct
GGDGSDQLL

SEQ ID NO: 32740 - protein, 9 aa, synthetic construct
GGDGSDQLV

SEQ ID NO: 32741 - protein, 9 aa, synthetic construct
GGDGSDQLW

SEQ ID NO: 32742 - protein, 9 aa, synthetic construct
GGDGSDQMD

SEQ ID NO: 32743 - protein, 9 aa, synthetic construct
GGDGSDQMF

SEQ ID NO: 32744 - protein, 9 aa, synthetic construct
GGDGSDQMR

SEQ ID NO: 32745 - protein, 9 aa, synthetic construct
GGDGSDRAV

SEQ ID NO: 32746 - protein, 9 aa, synthetic construct
GGDGSDRFI

SEQ ID NO: 32747 - protein, 9 aa, synthetic construct
GGDGSDRFL

SEQ ID NO: 32748 - protein, 9 aa, synthetic construct
GGDGSDRID

SEQ ID NO: 32749 - protein, 9 aa, synthetic construct
GGDGSDRIE

SEQ ID NO: 32750 - protein, 9 aa, synthetic construct
GGDGSDRLQ

SEQ ID NO: 32751 - protein, 9 aa, synthetic construct
GGDGSDRLR

SEQ ID NO: 32752 - protein, 9 aa, synthetic construct
GGDGSDQFV

SEQ ID NO: 32753 - protein, 9 aa, synthetic construct
GGDGSDNYY

SEQ ID NO: 32754 - protein, 9 aa, synthetic construct
GGDGSDLLQ

SEQ ID NO: 32755 - protein, 9 aa, synthetic construct
GGDGSDNYF

SEQ ID NO: 32756 - protein, 9 aa, synthetic construct
GGDGSDLMF

SEQ ID NO: 32757 - protein, 9 aa, synthetic construct
GGDGSDLML

SEQ ID NO: 32758 - protein, 9 aa, synthetic construct
GGDGSDLMS

SEQ ID NO: 32759 - protein, 9 aa, synthetic construct
GGDGSDLVA

SEQ ID NO: 32760 - protein, 9 aa, synthetic construct
GGDGSDLVD

SEQ ID NO: 32761 - protein, 9 aa, synthetic construct
GGDGSDLVF

SEQ ID NO: 32762 - protein, 9 aa, synthetic construct
GGDGSDLVV

SEQ ID NO: 32763 - protein, 9 aa, synthetic construct
GGDGSDMLD

SEQ ID NO: 32764 - protein, 9 aa, synthetic construct
GGDGSDMLK

SEQ ID NO: 32765 - protein, 9 aa, synthetic construct
GGDGSDMLV

SEQ ID NO: 32766 - protein, 9 aa, synthetic construct
GGDGSDMMS

SEQ ID NO: 32767 - protein, 9 aa, synthetic construct
GGDGSDNIF

SEQ ID NO: 32768 - protein, 9 aa, synthetic construct
GGDGSDNIS

SEQ ID NO: 32769 - protein, 9 aa, synthetic construct
GGDGSDNLD

SEQ ID NO: 32770 - protein, 9 aa, synthetic construct
GGDGSDNLR

SEQ ID NO: 32771 - protein, 9 aa, synthetic construct
GGDGSDNLW

SEQ ID NO: 32772 - protein, 9 aa, synthetic construct
GGDGSDNLY

SEQ ID NO: 32773 - protein, 9 aa, synthetic construct
GGDGIDSVW

SEQ ID NO: 32774 - protein, 9 aa, synthetic construct
GGDGIDSLW

SEQ ID NO: 32775 - protein, 9 aa, synthetic construct
GGAGTDRLY

SEQ ID NO: 32776 - protein, 9 aa, synthetic construct
GGDGADKIF

SEQ ID NO: 32777 - protein, 9 aa, synthetic construct
GGDGADIMI

SEQ ID NO: 32778 - protein, 9 aa, synthetic construct
GGDGADIMR

SEQ ID NO: 32779 - protein, 9 aa, synthetic construct
GGDGADIVV

SEQ ID NO: 32780 - protein, 9 aa, synthetic construct
GGDGADIVY

SEQ ID NO: 32781 - protein, 9 aa, synthetic construct
GGDGADIYV

SEQ ID NO: 32782 - protein, 9 aa, synthetic construct
GGDGADIYY

SEQ ID NO: 32783 - protein, 9 aa, synthetic construct
GGDGADKAS

SEQ ID NO: 32784 - protein, 9 aa, synthetic construct
GGDGADKFY

SEQ ID NO: 32785 - protein, 9 aa, synthetic construct
GGDGADKIV

SEQ ID NO: 32786 - protein, 9 aa, synthetic construct
GGDGADRFM

SEQ ID NO: 32787 - protein, 9 aa, synthetic construct
GGDGADKLG

SEQ ID NO: 32788 - protein, 9 aa, synthetic construct
GGDGADKLH

SEQ ID NO: 32789 - protein, 9 aa, synthetic construct
GGDGADKLR

SEQ ID NO: 32790 - protein, 9 aa, synthetic construct
GGDGADKMI

SEQ ID NO: 32791 - protein, 9 aa, synthetic construct
GGDGADKVW

SEQ ID NO: 32792 - protein, 9 aa, synthetic construct
GGDGADLAT

SEQ ID NO: 32793 - protein, 9 aa, synthetic construct
GGDGADLAY

SEQ ID NO: 32794 - protein, 9 aa, synthetic construct
GGDGADLFH

SEQ ID NO: 32795 - protein, 9 aa, synthetic construct
GGDGADIMH

SEQ ID NO: 32796 - protein, 9 aa, synthetic construct
GGDGADIMD

SEQ ID NO: 32797 - protein, 9 aa, synthetic construct
GGDGADILM

SEQ ID NO: 32798 - protein, 9 aa, synthetic construct
GGDGADILC

SEQ ID NO: 32799 - protein, 9 aa, synthetic construct
GGDGADGVY

SEQ ID NO: 32800 - protein, 9 aa, synthetic construct
GGDGADHFY

SEQ ID NO: 32801 - protein, 9 aa, synthetic construct
GGDGADHIE

SEQ ID NO: 32802 - protein, 9 aa, synthetic construct
GGDGADHLE

SEQ ID NO: 32803 - protein, 9 aa, synthetic construct
GGDGADHLR

SEQ ID NO: 32804 - protein, 9 aa, synthetic construct
GGDGADHLS

SEQ ID NO: 32805 - protein, 9 aa, synthetic construct
GGDGADHLV

SEQ ID NO: 32806 - protein, 9 aa, synthetic construct
GGDGADHME

SEQ ID NO: 32807 - protein, 9 aa, synthetic construct
GGDGADHVS

SEQ ID NO: 32808 - protein, 9 aa, synthetic construct
GGDGADIAY

SEQ ID NO: 32809 - protein, 9 aa, synthetic construct
GGDGADIFA

SEQ ID NO: 32810 - protein, 9 aa, synthetic construct
GGDGADIFE

SEQ ID NO: 32811 - protein, 9 aa, synthetic construct
GGDGADIFS

SEQ ID NO: 32812 - protein, 9 aa, synthetic construct
GGDGADIFW

SEQ ID NO: 32813 - protein, 9 aa, synthetic construct
GGDGADIIR

SEQ ID NO: 32814 - protein, 9 aa, synthetic construct
GGDGADIIT

SEQ ID NO: 32815 - protein, 9 aa, synthetic construct
GGDGADIIV

SEQ ID NO: 32816 - protein, 9 aa, synthetic construct
GGDGADLFY

SEQ ID NO: 32817 - protein, 9 aa, synthetic construct
GGDGADLIQ

SEQ ID NO: 32818 - protein, 9 aa, synthetic construct
GGDGADLLM

SEQ ID NO: 32819 - protein, 9 aa, synthetic construct
GGDGADNMR

SEQ ID NO: 32820 - protein, 9 aa, synthetic construct
GGDGADQAH

SEQ ID NO: 32821 - protein, 9 aa, synthetic construct
GGDGADQFR

SEQ ID NO: 32822 - protein, 9 aa, synthetic construct
GGDGADQFS

SEQ ID NO: 32823 - protein, 9 aa, synthetic construct
GGDGADQIA

SEQ ID NO: 32824 - protein, 9 aa, synthetic construct
GGDGADQIH

SEQ ID NO: 32825 - protein, 9 aa, synthetic construct
GGDGADQIN

SEQ ID NO: 32826 - protein, 9 aa, synthetic construct
GGDGADQIR

SEQ ID NO: 32827 - protein, 9 aa, synthetic construct
GGDGADQLA

SEQ ID NO: 32828 - protein, 9 aa, synthetic construct
GGDGADQLC

SEQ ID NO: 32829 - protein, 9 aa, synthetic construct
GGDGADQLG

SEQ ID NO: 32830 - protein, 9 aa, synthetic construct
GGDGADQMD

SEQ ID NO: 32831 - protein, 9 aa, synthetic construct
GGDGADQMQ

SEQ ID NO: 32832 - protein, 9 aa, synthetic construct
GGDGADQMY

SEQ ID NO: 32833 - protein, 9 aa, synthetic construct
GGDGADQVF

SEQ ID NO: 32834 - protein, 9 aa, synthetic construct
GGDGADQVT

SEQ ID NO: 32835 - protein, 9 aa, synthetic construct
GGDGADRAV

SEQ ID NO: 32836 - protein, 9 aa, synthetic construct
GGDGADRFA

SEQ ID NO: 32837 - protein, 9 aa, synthetic construct
GGDGADNVF

SEQ ID NO: 32838 - protein, 9 aa, synthetic construct
GGDGADNIR

SEQ ID NO: 32839 - protein, 9 aa, synthetic construct
GGDGADLLN

SEQ ID NO: 32840 - protein, 9 aa, synthetic construct
GGDGADNAG

SEQ ID NO: 32841 - protein, 9 aa, synthetic construct
GGDGADLME

SEQ ID NO: 32842 - protein, 9 aa, synthetic construct
GGDGADLMN

SEQ ID NO: 32843 - protein, 9 aa, synthetic construct
GGDGADLMR

SEQ ID NO: 32844 - protein, 9 aa, synthetic construct
GGDGADLMT

SEQ ID NO: 32845 - protein, 9 aa, synthetic construct
GGDGADLMV

SEQ ID NO: 32846 - protein, 9 aa, synthetic construct
GGDGADLVS

SEQ ID NO: 32847 - protein, 9 aa, synthetic construct
GGDGADLYY

SEQ ID NO: 32848 - protein, 9 aa, synthetic construct
GGDGADMIA

SEQ ID NO: 32849 - protein, 9 aa, synthetic construct
GGDGADMIR

SEQ ID NO: 32850 - protein, 9 aa, synthetic construct
GGDGADMIV

SEQ ID NO: 32851 - protein, 9 aa, synthetic construct
GGDGADMIW

SEQ ID NO: 32852 - protein, 9 aa, synthetic construct
GGDGADMIY

SEQ ID NO: 32853 - protein, 9 aa, synthetic construct
GGDGADMLE

SEQ ID NO: 32854 - protein, 9 aa, synthetic construct
GGDGADMLH

SEQ ID NO: 32855 - protein, 9 aa, synthetic construct
GGDGADMLI

SEQ ID NO: 32856 - protein, 9 aa, synthetic construct
GGDGADMLM

SEQ ID NO: 32857 - protein, 9 aa, synthetic construct
GGDGADMLN

SEQ ID NO: 32858 - protein, 9 aa, synthetic construct
GGDGADGLY

SEQ ID NO: 32859 - protein, 9 aa, synthetic construct
GGDGADGLT

SEQ ID NO: 32860 - protein, 9 aa, synthetic construct
GGDGADGLS

SEQ ID NO: 32861 - protein, 9 aa, synthetic construct
GGCGNDNIR

SEQ ID NO: 32862 - protein, 9 aa, synthetic construct
GGCGNDVLV

SEQ ID NO: 32863 - protein, 9 aa, synthetic construct
GGCGNDWMH

SEQ ID NO: 32864 - protein, 9 aa, synthetic construct
GGCGSDTLT

SEQ ID NO: 32865 - protein, 9 aa, synthetic construct
GGCGVDVLA

SEQ ID NO: 32866 - protein, 9 aa, synthetic construct
GGDGADAAY

SEQ ID NO: 32867 - protein, 9 aa, synthetic construct
GGDGADAIF

SEQ ID NO: 32868 - protein, 9 aa, synthetic construct
GGDGADAIH

SEQ ID NO: 32869 - protein, 9 aa, synthetic construct
GGDGADAIK

SEQ ID NO: 32870 - protein, 9 aa, synthetic construct
GGDGADAIS

SEQ ID NO: 32871 - protein, 9 aa, synthetic construct
GGDGADAIT

SEQ ID NO: 32872 - protein, 9 aa, synthetic construct
GGDGADAIV

SEQ ID NO: 32873 - protein, 9 aa, synthetic construct
GGDGADALA

SEQ ID NO: 32874 - protein, 9 aa, synthetic construct
GGDGADALK

SEQ ID NO: 32875 - protein, 9 aa, synthetic construct
GGDGADALR

SEQ ID NO: 32876 - protein, 9 aa, synthetic construct
GGDGADAMD

SEQ ID NO: 32877 - protein, 9 aa, synthetic construct
GGDGADAMG

SEQ ID NO: 32878 - protein, 9 aa, synthetic construct
GGDGADAMT

SEQ ID NO: 32879 - protein, 9 aa, synthetic construct
GGCGNDTLI

SEQ ID NO: 32880 - protein, 9 aa, synthetic construct
GGCGNDFLS

SEQ ID NO: 32881 - protein, 9 aa, synthetic construct
GGDGADCLL

SEQ ID NO: 32882 - protein, 9 aa, synthetic construct
GGCGEDLLF

SEQ ID NO: 32883 - protein, 9 aa, synthetic construct
GGAGYDYAV

SEQ ID NO: 32884 - protein, 9 aa, synthetic construct
GGAGYDYIE

SEQ ID NO: 32885 - protein, 9 aa, synthetic construct
GGAGYDYIH

SEQ ID NO: 32886 - protein, 9 aa, synthetic construct
GGAGYDYLT

SEQ ID NO: 32887 - protein, 9 aa, synthetic construct
GGAGYDYLV

SEQ ID NO: 32888 - protein, 9 aa, synthetic construct
GGAGYDYMS

SEQ ID NO: 32889 - protein, 9 aa, synthetic construct
GGBGADSID

SEQ ID NO: 32890 - protein, 9 aa, synthetic construct
GGCGADIFF

SEQ ID NO: 32891 - protein, 9 aa, synthetic construct
GGCGADTID

SEQ ID NO: 32892 - protein, 9 aa, synthetic construct
GGCGDDALA

SEQ ID NO: 32893 - protein, 9 aa, synthetic construct
GGCGDDDLS

SEQ ID NO: 32894 - protein, 9 aa, synthetic construct
GGCGDDEIH

SEQ ID NO: 32895 - protein, 9 aa, synthetic construct
GGCGDDIFE

SEQ ID NO: 32896 - protein, 9 aa, synthetic construct
GGCGDDQIT

SEQ ID NO: 32897 - protein, 9 aa, synthetic construct
GGCGDDSIS

SEQ ID NO: 32898 - protein, 9 aa, synthetic construct
GGCGDDTVR

SEQ ID NO: 32899 - protein, 9 aa, synthetic construct
GGCGDDYIN

SEQ ID NO: 32900 - protein, 9 aa, synthetic construct
GGDGADAVT

SEQ ID NO: 32901 - protein, 9 aa, synthetic construct
GGDGADDIQ

SEQ ID NO: 32902 - protein, 9 aa, synthetic construct
GGDGADGLR

SEQ ID NO: 32903 - protein, 9 aa, synthetic construct
GGDGADFAM

SEQ ID NO: 32904 - protein, 9 aa, synthetic construct
GGDGADFAV

SEQ ID NO: 32905 - protein, 9 aa, synthetic construct
GGDGADFFS

SEQ ID NO: 32906 - protein, 9 aa, synthetic construct
GGDGADFFT

SEQ ID NO: 32907 - protein, 9 aa, synthetic construct
GGDGADFIQ

SEQ ID NO: 32908 - protein, 9 aa, synthetic construct
GGDGADFIR

SEQ ID NO: 32909 - protein, 9 aa, synthetic construct
GGDGADFLG

SEQ ID NO: 32910 - protein, 9 aa, synthetic construct
GGDGADFLL

SEQ ID NO: 32911 - protein, 9 aa, synthetic construct
GGDGADFLQ

SEQ ID NO: 32912 - protein, 9 aa, synthetic construct
GGDGADFLR

SEQ ID NO: 32913 - protein, 9 aa, synthetic construct
GGDGADFLS

SEQ ID NO: 32914 - protein, 9 aa, synthetic construct
GGDGADFLT

SEQ ID NO: 32915 - protein, 9 aa, synthetic construct
GGDGADFLV

SEQ ID NO: 32916 - protein, 9 aa, synthetic construct
GGDGADFLW

SEQ ID NO: 32917 - protein, 9 aa, synthetic construct
GGDGADFVA

SEQ ID NO: 32918 - protein, 9 aa, synthetic construct
GGDGADFVE

SEQ ID NO: 32919 - protein, 9 aa, synthetic construct
GGDGADGLF

SEQ ID NO: 32920 - protein, 9 aa, synthetic construct
GGDGADGLI

SEQ ID NO: 32921 - protein, 9 aa, synthetic construct
GGDGADFAR

SEQ ID NO: 32922 - protein, 9 aa, synthetic construct
GGDGADEVS

SEQ ID NO: 32923 - protein, 9 aa, synthetic construct
GGDGADDLA

SEQ ID NO: 32924 - protein, 9 aa, synthetic construct
GGDGADEMH

SEQ ID NO: 32925 - protein, 9 aa, synthetic construct
GGDGADDLQ

SEQ ID NO: 32926 - protein, 9 aa, synthetic construct
GGDGADDLV

SEQ ID NO: 32927 - protein, 9 aa, synthetic construct
GGDGADDMH

SEQ ID NO: 32928 - protein, 9 aa, synthetic construct
GGDGADDMR

SEQ ID NO: 32929 - protein, 9 aa, synthetic construct
GGDGADDMT

SEQ ID NO: 32930 - protein, 9 aa, synthetic construct
GGDGADDVF

SEQ ID NO: 32931 - protein, 9 aa, synthetic construct
GGDGADDVV

SEQ ID NO: 32932 - protein, 9 aa, synthetic construct
GGDGADEAT

SEQ ID NO: 32933 - protein, 9 aa, synthetic construct
GGDGADEFD

SEQ ID NO: 32934 - protein, 9 aa, synthetic construct
GGDGADEFS

SEQ ID NO: 32935 - protein, 9 aa, synthetic construct
GGDGADEFV

SEQ ID NO: 32936 - protein, 9 aa, synthetic construct
GGDGADEID

SEQ ID NO: 32937 - protein, 9 aa, synthetic construct
GGDGADEIQ

SEQ ID NO: 32938 - protein, 9 aa, synthetic construct
GGDGADEIV

SEQ ID NO: 32939 - protein, 9 aa, synthetic construct
GGDGADELA

SEQ ID NO: 32940 - protein, 9 aa, synthetic construct
GGDGADELE

SEQ ID NO: 32941 - protein, 9 aa, synthetic construct
GGDGADELF

SEQ ID NO: 32942 - protein, 9 aa, synthetic construct
GGDGADRFL

SEQ ID NO: 32943 - protein, 9 aa, synthetic construct
GGDGADRFY

SEQ ID NO: 32944 - protein, 9 aa, synthetic construct
GGDGDDHLR

SEQ ID NO: 32945 - protein, 9 aa, synthetic construct
GGDGDDDLE

SEQ ID NO: 32946 - protein, 9 aa, synthetic construct
GGDGDDAVY

SEQ ID NO: 32947 - protein, 9 aa, synthetic construct
GGDGDDCLI

SEQ ID NO: 32948 - protein, 9 aa, synthetic construct
GGDGDDDAR

SEQ ID NO: 32949 - protein, 9 aa, synthetic construct
GGDGDDDFA

SEQ ID NO: 32950 - protein, 9 aa, synthetic construct
GGDGDDDIE

SEQ ID NO: 32951 - protein, 9 aa, synthetic construct
GGDGDDDIH

SEQ ID NO: 32952 - protein, 9 aa, synthetic construct
GGDGDDDIQ

SEQ ID NO: 32953 - protein, 9 aa, synthetic construct
GGDGDDDIW

SEQ ID NO: 32954 - protein, 9 aa, synthetic construct
GGDGDDDLK

SEQ ID NO: 32955 - protein, 9 aa, synthetic construct
GGDGADRIF

SEQ ID NO: 32956 - protein, 9 aa, synthetic construct
GGDGDDDVA

SEQ ID NO: 32957 - protein, 9 aa, synthetic construct
GGDGDDDVD

SEQ ID NO: 32958 - protein, 9 aa, synthetic construct
GGDGDDDVN

SEQ ID NO: 32959 - protein, 9 aa, synthetic construct
GGDGDDDVQ

SEQ ID NO: 32960 - protein, 9 aa, synthetic construct
GGDGDDDVR

SEQ ID NO: 32961 - protein, 9 aa, synthetic construct
GGDGDDDYF

SEQ ID NO: 32962 - protein, 9 aa, synthetic construct
GGDGDDDYV

SEQ ID NO: 32963 - protein, 9 aa, synthetic construct
GGDGDDEFV

SEQ ID NO: 32964 - protein, 9 aa, synthetic construct
GGDGDDAVT

SEQ ID NO: 32965 - protein, 9 aa, synthetic construct
GGDGDDAVS

SEQ ID NO: 32966 - protein, 9 aa, synthetic construct
GGDGDDAVQ

SEQ ID NO: 32967 - protein, 9 aa, synthetic construct
GGDGDDAVD

SEQ ID NO: 32968 - protein, 9 aa, synthetic construct
GGDGCDRVW

SEQ ID NO: 32969 - protein, 9 aa, synthetic construct
GGDGCDTAV

SEQ ID NO: 32970 - protein, 9 aa, synthetic construct
GGDGCDTIV

SEQ ID NO: 32971 - protein, 9 aa, synthetic construct
GGDGCDTLC

SEQ ID NO: 32972 - protein, 9 aa, synthetic construct
GGDGCDTLE

SEQ ID NO: 32973 - protein, 9 aa, synthetic construct
GGDGCDTLS

SEQ ID NO: 32974 - protein, 9 aa, synthetic construct
GGDGCDTVS

SEQ ID NO: 32975 - protein, 9 aa, synthetic construct
GGDGCDTVY

SEQ ID NO: 32976 - protein, 9 aa, synthetic construct
GGDGCDVLS

SEQ ID NO: 32977 - protein, 9 aa, synthetic construct
GGDGDDAAT

SEQ ID NO: 32978 - protein, 9 aa, synthetic construct
GGDGDDAFV

SEQ ID NO: 32979 - protein, 9 aa, synthetic construct
GGDGDDAIF

SEQ ID NO: 32980 - protein, 9 aa, synthetic construct
GGDGDDAIK

SEQ ID NO: 32981 - protein, 9 aa, synthetic construct
GGDGDDAIN

SEQ ID NO: 32982 - protein, 9 aa, synthetic construct
GGDGDDALA

SEQ ID NO: 32983 - protein, 9 aa, synthetic construct
GGDGDDALG

SEQ ID NO: 32984 - protein, 9 aa, synthetic construct
GGDGDDALM

SEQ ID NO: 32985 - protein, 9 aa, synthetic construct
GGDGDDEIE

SEQ ID NO: 32986 - protein, 9 aa, synthetic construct
GGDGDDEIN

SEQ ID NO: 32987 - protein, 9 aa, synthetic construct
GGDGDDEIS

SEQ ID NO: 32988 - protein, 9 aa, synthetic construct
GGDGDDGAY

SEQ ID NO: 32989 - protein, 9 aa, synthetic construct
GGDGDDGIR

SEQ ID NO: 32990 - protein, 9 aa, synthetic construct
GGDGDDGIS

SEQ ID NO: 32991 - protein, 9 aa, synthetic construct
GGDGDDGIW

SEQ ID NO: 32992 - protein, 9 aa, synthetic construct
GGDGDDGIY

SEQ ID NO: 32993 - protein, 9 aa, synthetic construct
GGDGDDGLD

SEQ ID NO: 32994 - protein, 9 aa, synthetic construct
GGDGDDGLE

SEQ ID NO: 32995 - protein, 9 aa, synthetic construct
GGDGDDGLQ

SEQ ID NO: 32996 - protein, 9 aa, synthetic construct
GGDGDDGLS

SEQ ID NO: 32997 - protein, 9 aa, synthetic construct
GGDGDDGLW

SEQ ID NO: 32998 - protein, 9 aa, synthetic construct
GGDGDDGMS

SEQ ID NO: 32999 - protein, 9 aa, synthetic construct
GGDGDDGVW

SEQ ID NO: 33000 - protein, 9 aa, synthetic construct
GGDGDDHFI

SEQ ID NO: 33001 - protein, 9 aa, synthetic construct
GGDGDDHFS

SEQ ID NO: 33002 - protein, 9 aa, synthetic construct
GGDGDDHIN

SEQ ID NO: 33003 - protein, 9 aa, synthetic construct
GGDGDDHIS

SEQ ID NO: 33004 - protein, 9 aa, synthetic construct
GGDGDDHLH

SEQ ID NO: 33005 - protein, 9 aa, synthetic construct
GGDGDDHLM

SEQ ID NO: 33006 - protein, 9 aa, synthetic construct
GGDGDDGID

SEQ ID NO: 33007 - protein, 9 aa, synthetic construct
GGDGDDFYI

SEQ ID NO: 33008 - protein, 9 aa, synthetic construct
GGDGDDEIT

SEQ ID NO: 33009 - protein, 9 aa, synthetic construct
GGDGDDFYG

SEQ ID NO: 33010 - protein, 9 aa, synthetic construct
GGDGDDELV

SEQ ID NO: 33011 - protein, 9 aa, synthetic construct
GGDGDDEMA

SEQ ID NO: 33012 - protein, 9 aa, synthetic construct
GGDGDDEMT

SEQ ID NO: 33013 - protein, 9 aa, synthetic construct
GGDGDDEVK

SEQ ID NO: 33014 - protein, 9 aa, synthetic construct
GGDGDDEVM

SEQ ID NO: 33015 - protein, 9 aa, synthetic construct
GGDGDDEVN

SEQ ID NO: 33016 - protein, 9 aa, synthetic construct
GGDGDDFAV

SEQ ID NO: 33017 - protein, 9 aa, synthetic construct
GGDGDDFAY

SEQ ID NO: 33018 - protein, 9 aa, synthetic construct
GGDGDDFFD

SEQ ID NO: 33019 - protein, 9 aa, synthetic construct
GGDGDDFFT

SEQ ID NO: 33020 - protein, 9 aa, synthetic construct
GGDGDDFIG

SEQ ID NO: 33021 - protein, 9 aa, synthetic construct
GGDGDDFII

SEQ ID NO: 33022 - protein, 9 aa, synthetic construct
GGDGDDFIM

SEQ ID NO: 33023 - protein, 9 aa, synthetic construct
GGDGDDFIQ

SEQ ID NO: 33024 - protein, 9 aa, synthetic construct
GGDGDDFMA

SEQ ID NO: 33025 - protein, 9 aa, synthetic construct
GGDGDDFVG

SEQ ID NO: 33026 - protein, 9 aa, synthetic construct
GGDGDDFVS

SEQ ID NO: 33027 - protein, 9 aa, synthetic construct
GGDGCDRLD

SEQ ID NO: 33028 - protein, 9 aa, synthetic construct
GGDGCDRLA

SEQ ID NO: 33029 - protein, 9 aa, synthetic construct
GGDGCDQIL

SEQ ID NO: 33030 - protein, 9 aa, synthetic construct
GGDGADSLP

SEQ ID NO: 33031 - protein, 9 aa, synthetic construct
GGDGADTAV

SEQ ID NO: 33032 - protein, 9 aa, synthetic construct
GGDGADTAW

SEQ ID NO: 33033 - protein, 9 aa, synthetic construct
GGDGADTFE

SEQ ID NO: 33034 - protein, 9 aa, synthetic construct
GGDGADTFH

SEQ ID NO: 33035 - protein, 9 aa, synthetic construct
GGDGADTFS

SEQ ID NO: 33036 - protein, 9 aa, synthetic construct
GGDGADTIK

SEQ ID NO: 33037 - protein, 9 aa, synthetic construct
GGDGADTIM

SEQ ID NO: 33038 - protein, 9 aa, synthetic construct
GGDGADTMN

SEQ ID NO: 33039 - protein, 9 aa, synthetic construct
GGDGADTMY

SEQ ID NO: 33040 - protein, 9 aa, synthetic construct
GGDGADTVQ

SEQ ID NO: 33041 - protein, 9 aa, synthetic construct
GGDGADTVV

SEQ ID NO: 33042 - protein, 9 aa, synthetic construct
GGDGADTYK

SEQ ID NO: 33043 - protein, 9 aa, synthetic construct
GGDGADTYR

SEQ ID NO: 33044 - protein, 9 aa, synthetic construct
GGDGADTYY

SEQ ID NO: 33045 - protein, 9 aa, synthetic construct
GGDGADVAF

SEQ ID NO: 33046 - protein, 9 aa, synthetic construct
GGDGADVFD

SEQ ID NO: 33047 - protein, 9 aa, synthetic construct
GGDGADVFE

SEQ ID NO: 33048 - protein, 9 aa, synthetic construct
GGDGADSVT

SEQ ID NO: 33049 - protein, 9 aa, synthetic construct
GGDGADSIK

SEQ ID NO: 33050 - protein, 9 aa, synthetic construct
GGDGADVFQ

SEQ ID NO: 33051 - protein, 9 aa, synthetic construct
GGDGADSIG

SEQ ID NO: 33052 - protein, 9 aa, synthetic construct
GGDGADRIG

SEQ ID NO: 33053 - protein, 9 aa, synthetic construct
GGDGADRIR

SEQ ID NO: 33054 - protein, 9 aa, synthetic construct
GGDGADRLG

SEQ ID NO: 33055 - protein, 9 aa, synthetic construct
GGDGADRLK

SEQ ID NO: 33056 - protein, 9 aa, synthetic construct
GGDGADRLM

SEQ ID NO: 33057 - protein, 9 aa, synthetic construct
GGDGADRMF

SEQ ID NO: 33058 - protein, 9 aa, synthetic construct
GGDGADRML

SEQ ID NO: 33059 - protein, 9 aa, synthetic construct
GGDGADRMT

SEQ ID NO: 33060 - protein, 9 aa, synthetic construct
GGDGADRMY

SEQ ID NO: 33061 - protein, 9 aa, synthetic construct
GGDGADRVD

SEQ ID NO: 33062 - protein, 9 aa, synthetic construct
GGDGADRVE

SEQ ID NO: 33063 - protein, 9 aa, synthetic construct
GGDGADRVF

SEQ ID NO: 33064 - protein, 9 aa, synthetic construct
GGDGADRYV

SEQ ID NO: 33065 - protein, 9 aa, synthetic construct
GGDGADSAF

SEQ ID NO: 33066 - protein, 9 aa, synthetic construct
GGDGADSFI

SEQ ID NO: 33067 - protein, 9 aa, synthetic construct
GGDGADSFQ

SEQ ID NO: 33068 - protein, 9 aa, synthetic construct
GGDGADSFS

SEQ ID NO: 33069 - protein, 9 aa, synthetic construct
GGDGADVFF

SEQ ID NO: 33070 - protein, 9 aa, synthetic construct
GGDGADVFS

SEQ ID NO: 33071 - protein, 9 aa, synthetic construct
GGDGCDLLN

SEQ ID NO: 33072 - protein, 9 aa, synthetic construct
GGDGADYAN

SEQ ID NO: 33073 - protein, 9 aa, synthetic construct
GGDGADYIN

SEQ ID NO: 33074 - protein, 9 aa, synthetic construct
GGDGADYIR

SEQ ID NO: 33075 - protein, 9 aa, synthetic construct
GGDGADYIV

SEQ ID NO: 33076 - protein, 9 aa, synthetic construct
GGDGADYLA

SEQ ID NO: 33077 - protein, 9 aa, synthetic construct
GGDGADYLE

SEQ ID NO: 33078 - protein, 9 aa, synthetic construct
GGDGADYLG

SEQ ID NO: 33079 - protein, 9 aa, synthetic construct
GGDGADYLI

SEQ ID NO: 33080 - protein, 9 aa, synthetic construct
GGDGADYLK

SEQ ID NO: 33081 - protein, 9 aa, synthetic construct
GGDGADYLV

SEQ ID NO: 33082 - protein, 9 aa, synthetic construct
GGDGADYLY

SEQ ID NO: 33083 - protein, 9 aa, synthetic construct
GGDGADYMD

SEQ ID NO: 33084 - protein, 9 aa, synthetic construct
GGDGADYVD

SEQ ID NO: 33085 - protein, 9 aa, synthetic construct
GGDGADYVT

SEQ ID NO: 33086 - protein, 9 aa, synthetic construct
GGDGADYVY

SEQ ID NO: 33087 - protein, 9 aa, synthetic construct
GGDGCDDIQ

SEQ ID NO: 33088 - protein, 9 aa, synthetic construct
GGDGCDLIY

SEQ ID NO: 33089 - protein, 9 aa, synthetic construct
GGDGCDLLD

SEQ ID NO: 33090 - protein, 9 aa, synthetic construct
GGDGADYIF

SEQ ID NO: 33091 - protein, 9 aa, synthetic construct
GGDGADWVF

SEQ ID NO: 33092 - protein, 9 aa, synthetic construct
GGDGADVLK

SEQ ID NO: 33093 - protein, 9 aa, synthetic construct
GGDGADWMD

SEQ ID NO: 33094 - protein, 9 aa, synthetic construct
GGDGADVMA

SEQ ID NO: 33095 - protein, 9 aa, synthetic construct
GGDGADVMD

SEQ ID NO: 33096 - protein, 9 aa, synthetic construct
GGDGADVMV

SEQ ID NO: 33097 - protein, 9 aa, synthetic construct
GGDGADVMY

SEQ ID NO: 33098 - protein, 9 aa, synthetic construct
GGDGADVVA

SEQ ID NO: 33099 - protein, 9 aa, synthetic construct
GGDGADVVD

SEQ ID NO: 33100 - protein, 9 aa, synthetic construct
GGDGADVVR

SEQ ID NO: 33101 - protein, 9 aa, synthetic construct
GGDGADVVT

SEQ ID NO: 33102 - protein, 9 aa, synthetic construct
GGDGADVYL

SEQ ID NO: 33103 - protein, 9 aa, synthetic construct
GGDGADWII

SEQ ID NO: 33104 - protein, 9 aa, synthetic construct
GGDGADWIQ

SEQ ID NO: 33105 - protein, 9 aa, synthetic construct
GGDGADWIT

SEQ ID NO: 33106 - protein, 9 aa, synthetic construct
GGDGADWLL

SEQ ID NO: 33107 - protein, 9 aa, synthetic construct
GGDGADWLN

SEQ ID NO: 33108 - protein, 9 aa, synthetic construct
GGDGADWLT

SEQ ID NO: 33109 - protein, 9 aa, synthetic construct
GGDGADWLW

SEQ ID NO: 33110 - protein, 9 aa, synthetic construct
GGDGADWLY

SEQ ID NO: 33111 - protein, 9 aa, synthetic construct
GGAGYDWLL

SEQ ID NO: 33112 - protein, 9 aa, synthetic construct
GGAGYDVVV

SEQ ID NO: 33113 - protein, 9 aa, synthetic construct
GGAGYDVMN

SEQ ID NO: 33114 - protein, 9 aa, synthetic construct
GGAGVDIMN

SEQ ID NO: 33115 - protein, 9 aa, synthetic construct
GGAGVDIFC

SEQ ID NO: 33116 - protein, 9 aa, synthetic construct
GGAGVDIFR

SEQ ID NO: 33117 - protein, 9 aa, synthetic construct
GGAGVDIIS

SEQ ID NO: 33118 - protein, 9 aa, synthetic construct
GGAGVDIIT

SEQ ID NO: 33119 - protein, 9 aa, synthetic construct
GGAGVDIIY

SEQ ID NO: 33120 - protein, 9 aa, synthetic construct
GGAGVDILG

SEQ ID NO: 33121 - protein, 9 aa, synthetic construct
GGAGVDILQ

SEQ ID NO: 33122 - protein, 9 aa, synthetic construct
GGAGVDILY

SEQ ID NO: 33123 - protein, 9 aa, synthetic construct
GGAGVDIVL

SEQ ID NO: 33124 - protein, 9 aa, synthetic construct
GGAGYDVLY

SEQ ID NO: 33125 - protein, 9 aa, synthetic construct
GGAGVDIVR

SEQ ID NO: 33126 - protein, 9 aa, synthetic construct
GGAGVDKFL

SEQ ID NO: 33127 - protein, 9 aa, synthetic construct
GGAGVDKFY

SEQ ID NO: 33128 - protein, 9 aa, synthetic construct
GGAGVDKIE

SEQ ID NO: 33129 - protein, 9 aa, synthetic construct
GGAGVDKIF

SEQ ID NO: 33130 - protein, 9 aa, synthetic construct
GGAGVDKLD

SEQ ID NO: 33131 - protein, 9 aa, synthetic construct
GGAGVDKLN

SEQ ID NO: 33132 - protein, 9 aa, synthetic construct
GGAGVDKLQ

SEQ ID NO: 33133 - protein, 9 aa, synthetic construct
GGAGVDIAV

SEQ ID NO: 33134 - protein, 9 aa, synthetic construct
GGAGVDIAT

SEQ ID NO: 33135 - protein, 9 aa, synthetic construct
GGAGVDIAE

SEQ ID NO: 33136 - protein, 9 aa, synthetic construct
GGAGVDHMI

SEQ ID NO: 33137 - protein, 9 aa, synthetic construct
GGAGVDFIY

SEQ ID NO: 33138 - protein, 9 aa, synthetic construct
GGAGVDFLQ

SEQ ID NO: 33139 - protein, 9 aa, synthetic construct
GGAGVDFLS

SEQ ID NO: 33140 - protein, 9 aa, synthetic construct
GGAGVDFLY

SEQ ID NO: 33141 - protein, 9 aa, synthetic construct
GGAGVDFMR

SEQ ID NO: 33142 - protein, 9 aa, synthetic construct
GGAGVDFVL

SEQ ID NO: 33143 - protein, 9 aa, synthetic construct
GGAGVDGIL

SEQ ID NO: 33144 - protein, 9 aa, synthetic construct
GGAGVDGMS

SEQ ID NO: 33145 - protein, 9 aa, synthetic construct
GGAGVDHFF

SEQ ID NO: 33146 - protein, 9 aa, synthetic construct
GGAGVDHII

SEQ ID NO: 33147 - protein, 9 aa, synthetic construct
GGAGVDHIS

SEQ ID NO: 33148 - protein, 9 aa, synthetic construct
GGAGVDHIY

SEQ ID NO: 33149 - protein, 9 aa, synthetic construct
GGAGVDHLE

SEQ ID NO: 33150 - protein, 9 aa, synthetic construct
GGAGVDHLS

SEQ ID NO: 33151 - protein, 9 aa, synthetic construct
GGAGVDHLT

SEQ ID NO: 33152 - protein, 9 aa, synthetic construct
GGAGVDHLY

SEQ ID NO: 33153 - protein, 9 aa, synthetic construct
GGAGVDHME

SEQ ID NO: 33154 - protein, 9 aa, synthetic construct
GGAGVDKMF

SEQ ID NO: 33155 - protein, 9 aa, synthetic construct
GGAGVDKMT

SEQ ID NO: 33156 - protein, 9 aa, synthetic construct
GGAGVDKVQ

SEQ ID NO: 33157 - protein, 9 aa, synthetic construct
GGAGVDNLQ

SEQ ID NO: 33158 - protein, 9 aa, synthetic construct
GGAGVDNLV

SEQ ID NO: 33159 - protein, 9 aa, synthetic construct
GGAGVDNLW

SEQ ID NO: 33160 - protein, 9 aa, synthetic construct
GGAGVDNMT

SEQ ID NO: 33161 - protein, 9 aa, synthetic construct
GGAGVDQIN

SEQ ID NO: 33162 - protein, 9 aa, synthetic construct
GGAGVDQIY

SEQ ID NO: 33163 - protein, 9 aa, synthetic construct
GGAGVDQLA

SEQ ID NO: 33164 - protein, 9 aa, synthetic construct
GGAGVDQLE

SEQ ID NO: 33165 - protein, 9 aa, synthetic construct
GGAGVDQLI

SEQ ID NO: 33166 - protein, 9 aa, synthetic construct
GGAGVDQMF

SEQ ID NO: 33167 - protein, 9 aa, synthetic construct
GGAGVDQMI

SEQ ID NO: 33168 - protein, 9 aa, synthetic construct
GGAGVDRAI

SEQ ID NO: 33169 - protein, 9 aa, synthetic construct
GGAGVDRFT

SEQ ID NO: 33170 - protein, 9 aa, synthetic construct
GGAGVDRID

SEQ ID NO: 33171 - protein, 9 aa, synthetic construct
GGAGVDRIF

SEQ ID NO: 33172 - protein, 9 aa, synthetic construct
GGAGVDRIQ

SEQ ID NO: 33173 - protein, 9 aa, synthetic construct
GGAGVDRIW

SEQ ID NO: 33174 - protein, 9 aa, synthetic construct
GGAGVDRIY

SEQ ID NO: 33175 - protein, 9 aa, synthetic construct
GGAGVDNLS

SEQ ID NO: 33176 - protein, 9 aa, synthetic construct
GGAGVDNIS

SEQ ID NO: 33177 - protein, 9 aa, synthetic construct
GGAGVDKVS

SEQ ID NO: 33178 - protein, 9 aa, synthetic construct
GGAGVDNID

SEQ ID NO: 33179 - protein, 9 aa, synthetic construct
GGAGVDLFV

SEQ ID NO: 33180 - protein, 9 aa, synthetic construct
GGAGVDLIE

SEQ ID NO: 33181 - protein, 9 aa, synthetic construct
GGAGVDLIL

SEQ ID NO: 33182 - protein, 9 aa, synthetic construct
GGAGVDLIY

SEQ ID NO: 33183 - protein, 9 aa, synthetic construct
GGAGVDLLN

SEQ ID NO: 33184 - protein, 9 aa, synthetic construct
GGAGVDLLQ

SEQ ID NO: 33185 - protein, 9 aa, synthetic construct
GGAGVDLLV

SEQ ID NO: 33186 - protein, 9 aa, synthetic construct
GGAGVDLMV

SEQ ID NO: 33187 - protein, 9 aa, synthetic construct
GGAGVDLVG

SEQ ID NO: 33188 - protein, 9 aa, synthetic construct
GGAGVDLVS

SEQ ID NO: 33189 - protein, 9 aa, synthetic construct
GGAGVDMAR

SEQ ID NO: 33190 - protein, 9 aa, synthetic construct
GGAGVDMAS

SEQ ID NO: 33191 - protein, 9 aa, synthetic construct
GGAGVDMLM

SEQ ID NO: 33192 - protein, 9 aa, synthetic construct
GGAGVDMMD

SEQ ID NO: 33193 - protein, 9 aa, synthetic construct
GGAGVDMMI

SEQ ID NO: 33194 - protein, 9 aa, synthetic construct
GGAGVDMVV

SEQ ID NO: 33195 - protein, 9 aa, synthetic construct
GGAGVDMVY

SEQ ID NO: 33196 - protein, 9 aa, synthetic construct
GGAGVDEMR

SEQ ID NO: 33197 - protein, 9 aa, synthetic construct
GGAGVDEML

SEQ ID NO: 33198 - protein, 9 aa, synthetic construct
GGAGVDELR

SEQ ID NO: 33199 - protein, 9 aa, synthetic construct
GGAGTDTAL

SEQ ID NO: 33200 - protein, 9 aa, synthetic construct
GGAGTDTAQ

SEQ ID NO: 33201 - protein, 9 aa, synthetic construct
GGAGTDTFQ

SEQ ID NO: 33202 - protein, 9 aa, synthetic construct
GGAGTDTFR

SEQ ID NO: 33203 - protein, 9 aa, synthetic construct
GGAGTDTIY

SEQ ID NO: 33204 - protein, 9 aa, synthetic construct
GGAGTDTME

SEQ ID NO: 33205 - protein, 9 aa, synthetic construct
GGAGTDTMQ

SEQ ID NO: 33206 - protein, 9 aa, synthetic construct
GGAGTDTYI

SEQ ID NO: 33207 - protein, 9 aa, synthetic construct
GGAGTDTYL

SEQ ID NO: 33208 - protein, 9 aa, synthetic construct
GGAGTDTYR

SEQ ID NO: 33209 - protein, 9 aa, synthetic construct
GGAGTDVAN

SEQ ID NO: 33210 - protein, 9 aa, synthetic construct
GGAGTDVAR

SEQ ID NO: 33211 - protein, 9 aa, synthetic construct
GGAGTDVFA

SEQ ID NO: 33212 - protein, 9 aa, synthetic construct
GGAGTDVFV

SEQ ID NO: 33213 - protein, 9 aa, synthetic construct
GGAGTDVIE

SEQ ID NO: 33214 - protein, 9 aa, synthetic construct
GGAGTDVIN

SEQ ID NO: 33215 - protein, 9 aa, synthetic construct
GGAGTDVLE

SEQ ID NO: 33216 - protein, 9 aa, synthetic construct
GGAGTDVLR

SEQ ID NO: 33217 - protein, 9 aa, synthetic construct
GGAGTDTAM

SEQ ID NO: 33218 - protein, 9 aa, synthetic construct
GGAGTDTAH

SEQ ID NO: 33219 - protein, 9 aa, synthetic construct
GGAGTDVMD

SEQ ID NO: 33220 - protein, 9 aa, synthetic construct
GGAGTDSVV

SEQ ID NO: 33221 - protein, 9 aa, synthetic construct
GGAGTDRME

SEQ ID NO: 33222 - protein, 9 aa, synthetic construct
GGAGTDRMQ

SEQ ID NO: 33223 - protein, 9 aa, synthetic construct
GGAGTDRMS

SEQ ID NO: 33224 - protein, 9 aa, synthetic construct
GGAGTDRMV

SEQ ID NO: 33225 - protein, 9 aa, synthetic construct
GGAGTDRVN

SEQ ID NO: 33226 - protein, 9 aa, synthetic construct
GGAGTDRVR

SEQ ID NO: 33227 - protein, 9 aa, synthetic construct
GGAGTDRVV

SEQ ID NO: 33228 - protein, 9 aa, synthetic construct
GGAGTDSAR

SEQ ID NO: 33229 - protein, 9 aa, synthetic construct
GGAGTDSAV

SEQ ID NO: 33230 - protein, 9 aa, synthetic construct
GGAGTDSFA

SEQ ID NO: 33231 - protein, 9 aa, synthetic construct
GGAGTDSFL

SEQ ID NO: 33232 - protein, 9 aa, synthetic construct
GGAGTDSIA

SEQ ID NO: 33233 - protein, 9 aa, synthetic construct
GGAGTDSIQ

SEQ ID NO: 33234 - protein, 9 aa, synthetic construct
GGAGTDSIR

SEQ ID NO: 33235 - protein, 9 aa, synthetic construct
GGAGTDSMA

SEQ ID NO: 33236 - protein, 9 aa, synthetic construct
GGAGTDSMI

SEQ ID NO: 33237 - protein, 9 aa, synthetic construct
GGAGTDSVD

SEQ ID NO: 33238 - protein, 9 aa, synthetic construct
GGAGTDVLS

SEQ ID NO: 33239 - protein, 9 aa, synthetic construct
GGAGTDVMI

SEQ ID NO: 33240 - protein, 9 aa, synthetic construct
GGAGVDELL

SEQ ID NO: 33241 - protein, 9 aa, synthetic construct
GGAGVDAAI

SEQ ID NO: 33242 - protein, 9 aa, synthetic construct
GGAGVDAFV

SEQ ID NO: 33243 - protein, 9 aa, synthetic construct
GGAGVDAFY

SEQ ID NO: 33244 - protein, 9 aa, synthetic construct
GGAGVDALK

SEQ ID NO: 33245 - protein, 9 aa, synthetic construct
GGAGVDALQ

SEQ ID NO: 33246 - protein, 9 aa, synthetic construct
GGAGVDAMS

SEQ ID NO: 33247 - protein, 9 aa, synthetic construct
GGAGVDAMT

SEQ ID NO: 33248 - protein, 9 aa, synthetic construct
GGAGVDAVL

SEQ ID NO: 33249 - protein, 9 aa, synthetic construct
GGAGVDCVA

SEQ ID NO: 33250 - protein, 9 aa, synthetic construct
GGAGVDDIN

SEQ ID NO: 33251 - protein, 9 aa, synthetic construct
GGAGVDDIQ

SEQ ID NO: 33252 - protein, 9 aa, synthetic construct
GGAGVDDLI

SEQ ID NO: 33253 - protein, 9 aa, synthetic construct
GGAGVDDLR

SEQ ID NO: 33254 - protein, 9 aa, synthetic construct
GGAGVDDLS

SEQ ID NO: 33255 - protein, 9 aa, synthetic construct
GGAGVDDMI

SEQ ID NO: 33256 - protein, 9 aa, synthetic construct
GGAGVDELD

SEQ ID NO: 33257 - protein, 9 aa, synthetic construct
GGAGVDELE

SEQ ID NO: 33258 - protein, 9 aa, synthetic construct
GGAGVDELK

SEQ ID NO: 33259 - protein, 9 aa, synthetic construct
GGAGVDAAV

SEQ ID NO: 33260 - protein, 9 aa, synthetic construct
GGAGTDYMT

SEQ ID NO: 33261 - protein, 9 aa, synthetic construct
GGAGTDVMY

SEQ ID NO: 33262 - protein, 9 aa, synthetic construct
GGAGTDYLV

SEQ ID NO: 33263 - protein, 9 aa, synthetic construct
GGAGTDVVF

SEQ ID NO: 33264 - protein, 9 aa, synthetic construct
GGAGTDVVM

SEQ ID NO: 33265 - protein, 9 aa, synthetic construct
GGAGTDVVQ

SEQ ID NO: 33266 - protein, 9 aa, synthetic construct
GGAGTDVYF

SEQ ID NO: 33267 - protein, 9 aa, synthetic construct
GGAGTDWAA

SEQ ID NO: 33268 - protein, 9 aa, synthetic construct
GGAGTDWAF

SEQ ID NO: 33269 - protein, 9 aa, synthetic construct
GGAGTDWAL

SEQ ID NO: 33270 - protein, 9 aa, synthetic construct
GGAGTDWAS

SEQ ID NO: 33271 - protein, 9 aa, synthetic construct
GGAGTDWIW

SEQ ID NO: 33272 - protein, 9 aa, synthetic construct
GGAGTDYAA

SEQ ID NO: 33273 - protein, 9 aa, synthetic construct
GGAGTDYAF

SEQ ID NO: 33274 - protein, 9 aa, synthetic construct
GGAGTDYAQ

SEQ ID NO: 33275 - protein, 9 aa, synthetic construct
GGAGTDYFQ

SEQ ID NO: 33276 - protein, 9 aa, synthetic construct
GGAGTDYLA

SEQ ID NO: 33277 - protein, 9 aa, synthetic construct
GGAGTDYLK

SEQ ID NO: 33278 - protein, 9 aa, synthetic construct
GGAGTDYLL

SEQ ID NO: 33279 - protein, 9 aa, synthetic construct
GGAGTDYLT

SEQ ID NO: 33280 - protein, 9 aa, synthetic construct
GGAGVDRLW

SEQ ID NO: 33281 - protein, 9 aa, synthetic construct
GGAGVDRML

SEQ ID NO: 33282 - protein, 9 aa, synthetic construct
GGAGVDSAD

SEQ ID NO: 33283 - protein, 9 aa, synthetic construct
GGAGYDHIF

SEQ ID NO: 33284 - protein, 9 aa, synthetic construct
GGAGYDHLY

SEQ ID NO: 33285 - protein, 9 aa, synthetic construct
GGAGYDILA

SEQ ID NO: 33286 - protein, 9 aa, synthetic construct
GGAGYDILS

SEQ ID NO: 33287 - protein, 9 aa, synthetic construct
GGAGYDILT

SEQ ID NO: 33288 - protein, 9 aa, synthetic construct
GGAGYDILY

SEQ ID NO: 33289 - protein, 9 aa, synthetic construct
GGAGYDIVR

SEQ ID NO: 33290 - protein, 9 aa, synthetic construct
GGAGYDIYL

SEQ ID NO: 33291 - protein, 9 aa, synthetic construct
GGAGYDKIS

SEQ ID NO: 33292 - protein, 9 aa, synthetic construct
GGAGYDLLI

SEQ ID NO: 33293 - protein, 9 aa, synthetic construct
GGAGYDLLQ

SEQ ID NO: 33294 - protein, 9 aa, synthetic construct
GGAGYDLLR

SEQ ID NO: 33295 - protein, 9 aa, synthetic construct
GGAGYDLLV

SEQ ID NO: 33296 - protein, 9 aa, synthetic construct
GGAGYDLLY

SEQ ID NO: 33297 - protein, 9 aa, synthetic construct
GGAGYDLVR

SEQ ID NO: 33298 - protein, 9 aa, synthetic construct
GGAGYDMAL

SEQ ID NO: 33299 - protein, 9 aa, synthetic construct
GGAGYDMLY

SEQ ID NO: 33300 - protein, 9 aa, synthetic construct
GGAGYDNLH

SEQ ID NO: 33301 - protein, 9 aa, synthetic construct
GGAGYDHLD

SEQ ID NO: 33302 - protein, 9 aa, synthetic construct
GGAGYDGLL

SEQ ID NO: 33303 - protein, 9 aa, synthetic construct
GGAGYDQIS

SEQ ID NO: 33304 - protein, 9 aa, synthetic construct
GGAGYDFLE

SEQ ID NO: 33305 - protein, 9 aa, synthetic construct
GGAGWDVAH

SEQ ID NO: 33306 - protein, 9 aa, synthetic construct
GGAGWDVFH

SEQ ID NO: 33307 - protein, 9 aa, synthetic construct
GGAGWDVLA

SEQ ID NO: 33308 - protein, 9 aa, synthetic construct
GGAGWDYLD

SEQ ID NO: 33309 - protein, 9 aa, synthetic construct
GGAGXDLAN

SEQ ID NO: 33310 - protein, 9 aa, synthetic construct
GGAGXDSLF

SEQ ID NO: 33311 - protein, 9 aa, synthetic construct
GGAGXDTIE

SEQ ID NO: 33312 - protein, 9 aa, synthetic construct
GGAGXDTLS

SEQ ID NO: 33313 - protein, 9 aa, synthetic construct
GGAGYDAIW

SEQ ID NO: 33314 - protein, 9 aa, synthetic construct
GGAGYDALE

SEQ ID NO: 33315 - protein, 9 aa, synthetic construct
GGAGYDALF

SEQ ID NO: 33316 - protein, 9 aa, synthetic construct
GGAGYDALL

SEQ ID NO: 33317 - protein, 9 aa, synthetic construct
GGAGYDALM

SEQ ID NO: 33318 - protein, 9 aa, synthetic construct
GGAGYDAYI

SEQ ID NO: 33319 - protein, 9 aa, synthetic construct
GGAGYDAYY

SEQ ID NO: 33320 - protein, 9 aa, synthetic construct
GGAGYDELS

SEQ ID NO: 33321 - protein, 9 aa, synthetic construct
GGAGYDFLA

SEQ ID NO: 33322 - protein, 9 aa, synthetic construct
GGAGYDQIQ

SEQ ID NO: 33323 - protein, 9 aa, synthetic construct
GGAGYDQLL

SEQ ID NO: 33324 - protein, 9 aa, synthetic construct
GGAGWDTMN

SEQ ID NO: 33325 - protein, 9 aa, synthetic construct
GGAGYDTLF

SEQ ID NO: 33326 - protein, 9 aa, synthetic construct
GGAGYDTLI

SEQ ID NO: 33327 - protein, 9 aa, synthetic construct
GGAGYDTLM

SEQ ID NO: 33328 - protein, 9 aa, synthetic construct
GGAGYDTLR

SEQ ID NO: 33329 - protein, 9 aa, synthetic construct
GGAGYDTLS

SEQ ID NO: 33330 - protein, 9 aa, synthetic construct
GGAGYDTLV

SEQ ID NO: 33331 - protein, 9 aa, synthetic construct
GGAGYDTMI

SEQ ID NO: 33332 - protein, 9 aa, synthetic construct
GGAGYDTYF

SEQ ID NO: 33333 - protein, 9 aa, synthetic construct
GGAGYDTYY

SEQ ID NO: 33334 - protein, 9 aa, synthetic construct
GGAGYDVAL

SEQ ID NO: 33335 - protein, 9 aa, synthetic construct
GGAGYDVAV

SEQ ID NO: 33336 - protein, 9 aa, synthetic construct
GGAGYDVFH

SEQ ID NO: 33337 - protein, 9 aa, synthetic construct
GGAGYDVFR

SEQ ID NO: 33338 - protein, 9 aa, synthetic construct
GGAGYDVFV

SEQ ID NO: 33339 - protein, 9 aa, synthetic construct
GGAGYDVIY

SEQ ID NO: 33340 - protein, 9 aa, synthetic construct
GGAGYDVLE

SEQ ID NO: 33341 - protein, 9 aa, synthetic construct
GGAGYDVLK

SEQ ID NO: 33342 - protein, 9 aa, synthetic construct
GGAGYDVLN

SEQ ID NO: 33343 - protein, 9 aa, synthetic construct
GGAGYDTLH

SEQ ID NO: 33344 - protein, 9 aa, synthetic construct
GGAGYDTFV

SEQ ID NO: 33345 - protein, 9 aa, synthetic construct
GGAGYDQLS

SEQ ID NO: 33346 - protein, 9 aa, synthetic construct
GGAGYDTAY

SEQ ID NO: 33347 - protein, 9 aa, synthetic construct
GGAGYDQLT

SEQ ID NO: 33348 - protein, 9 aa, synthetic construct
GGAGYDQVN

SEQ ID NO: 33349 - protein, 9 aa, synthetic construct
GGAGYDRFV

SEQ ID NO: 33350 - protein, 9 aa, synthetic construct
GGAGYDRIY

SEQ ID NO: 33351 - protein, 9 aa, synthetic construct
GGAGYDRLA

SEQ ID NO: 33352 - protein, 9 aa, synthetic construct
GGAGYDRLD

SEQ ID NO: 33353 - protein, 9 aa, synthetic construct
GGAGYDRLF

SEQ ID NO: 33354 - protein, 9 aa, synthetic construct
GGAGYDRLS

SEQ ID NO: 33355 - protein, 9 aa, synthetic construct
GGAGYDSIR

SEQ ID NO: 33356 - protein, 9 aa, synthetic construct
GGAGYDSIW

SEQ ID NO: 33357 - protein, 9 aa, synthetic construct
GGAGYDSLL

SEQ ID NO: 33358 - protein, 9 aa, synthetic construct
GGAGYDSLT

SEQ ID NO: 33359 - protein, 9 aa, synthetic construct
GGAGYDSLV

SEQ ID NO: 33360 - protein, 9 aa, synthetic construct
GGAGYDTAD

SEQ ID NO: 33361 - protein, 9 aa, synthetic construct
GGAGYDTAI

SEQ ID NO: 33362 - protein, 9 aa, synthetic construct
GGAGYDTAL

SEQ ID NO: 33363 - protein, 9 aa, synthetic construct
GGAGYDTAV

SEQ ID NO: 33364 - protein, 9 aa, synthetic construct
GGAGWDTMT

SEQ ID NO: 33365 - protein, 9 aa, synthetic construct
GGAGWDTMI

SEQ ID NO: 33366 - protein, 9 aa, synthetic construct
GGAGVDSAE

SEQ ID NO: 33367 - protein, 9 aa, synthetic construct
GGAGVDTFN

SEQ ID NO: 33368 - protein, 9 aa, synthetic construct
GGAGVDTIL

SEQ ID NO: 33369 - protein, 9 aa, synthetic construct
GGAGVDTIQ

SEQ ID NO: 33370 - protein, 9 aa, synthetic construct
GGAGVDTLW

SEQ ID NO: 33371 - protein, 9 aa, synthetic construct
GGAGVDTMF

SEQ ID NO: 33372 - protein, 9 aa, synthetic construct
GGAGVDTML

SEQ ID NO: 33373 - protein, 9 aa, synthetic construct
GGAGVDTMN

SEQ ID NO: 33374 - protein, 9 aa, synthetic construct
GGAGVDTMQ

SEQ ID NO: 33375 - protein, 9 aa, synthetic construct
GGAGVDTVE

SEQ ID NO: 33376 - protein, 9 aa, synthetic construct
GGAGVDTYN

SEQ ID NO: 33377 - protein, 9 aa, synthetic construct
GGAGVDVAI

SEQ ID NO: 33378 - protein, 9 aa, synthetic construct
GGAGVDVAV

SEQ ID NO: 33379 - protein, 9 aa, synthetic construct
GGAGVDVFG

SEQ ID NO: 33380 - protein, 9 aa, synthetic construct
GGAGVDVIE

SEQ ID NO: 33381 - protein, 9 aa, synthetic construct
GGAGVDVIV

SEQ ID NO: 33382 - protein, 9 aa, synthetic construct
GGAGVDVIY

SEQ ID NO: 33383 - protein, 9 aa, synthetic construct
GGAGVDVLD

SEQ ID NO: 33384 - protein, 9 aa, synthetic construct
GGAGVDVLV

SEQ ID NO: 33385 - protein, 9 aa, synthetic construct
GGAGVDTFT

SEQ ID NO: 33386 - protein, 9 aa, synthetic construct
GGAGVDTFF

SEQ ID NO: 33387 - protein, 9 aa, synthetic construct
GGAGVDVVY

SEQ ID NO: 33388 - protein, 9 aa, synthetic construct
GGAGVDTFA

SEQ ID NO: 33389 - protein, 9 aa, synthetic construct
GGAGVDSAV

SEQ ID NO: 33390 - protein, 9 aa, synthetic construct
GGAGVDSFL

SEQ ID NO: 33391 - protein, 9 aa, synthetic construct
GGAGVDSIF

SEQ ID NO: 33392 - protein, 9 aa, synthetic construct
GGAGVDSIL

SEQ ID NO: 33393 - protein, 9 aa, synthetic construct
GGAGVDSIQ

SEQ ID NO: 33394 - protein, 9 aa, synthetic construct
GGAGVDSLE

SEQ ID NO: 33395 - protein, 9 aa, synthetic construct
GGAGVDSLY

SEQ ID NO: 33396 - protein, 9 aa, synthetic construct
GGAGVDSMA

SEQ ID NO: 33397 - protein, 9 aa, synthetic construct
GGAGVDSME

SEQ ID NO: 33398 - protein, 9 aa, synthetic construct
GGAGVDSMF

SEQ ID NO: 33399 - protein, 9 aa, synthetic construct
GGAGVDSMT

SEQ ID NO: 33400 - protein, 9 aa, synthetic construct
GGAGVDSMW

SEQ ID NO: 33401 - protein, 9 aa, synthetic construct
GGAGVDSVN

SEQ ID NO: 33402 - protein, 9 aa, synthetic construct
GGAGVDTAL

SEQ ID NO: 33403 - protein, 9 aa, synthetic construct
GGAGVDTAM

SEQ ID NO: 33404 - protein, 9 aa, synthetic construct
GGAGVDTAT

SEQ ID NO: 33405 - protein, 9 aa, synthetic construct
GGAGVDTAY

SEQ ID NO: 33406 - protein, 9 aa, synthetic construct
GGAGVDVMS

SEQ ID NO: 33407 - protein, 9 aa, synthetic construct
GGAGVDWAD

SEQ ID NO: 33408 - protein, 9 aa, synthetic construct
GGAGWDTLY

SEQ ID NO: 33409 - protein, 9 aa, synthetic construct
GGAGWDILN

SEQ ID NO: 33410 - protein, 9 aa, synthetic construct
GGAGWDNFV

SEQ ID NO: 33411 - protein, 9 aa, synthetic construct
GGAGWDNLF

SEQ ID NO: 33412 - protein, 9 aa, synthetic construct
GGAGWDNLR

SEQ ID NO: 33413 - protein, 9 aa, synthetic construct
GGAGWDNLT

SEQ ID NO: 33414 - protein, 9 aa, synthetic construct
GGAGWDQIF

SEQ ID NO: 33415 - protein, 9 aa, synthetic construct
GGAGWDQLK

SEQ ID NO: 33416 - protein, 9 aa, synthetic construct
GGAGWDQLR

SEQ ID NO: 33417 - protein, 9 aa, synthetic construct
GGAGWDRYH

SEQ ID NO: 33418 - protein, 9 aa, synthetic construct
GGAGWDSLD

SEQ ID NO: 33419 - protein, 9 aa, synthetic construct
GGAGWDTAI

SEQ ID NO: 33420 - protein, 9 aa, synthetic construct
GGAGWDTAT

SEQ ID NO: 33421 - protein, 9 aa, synthetic construct
GGAGWDTFD

SEQ ID NO: 33422 - protein, 9 aa, synthetic construct
GGAGWDTIS

SEQ ID NO: 33423 - protein, 9 aa, synthetic construct
GGAGWDTLK

SEQ ID NO: 33424 - protein, 9 aa, synthetic construct
GGAGWDTLM

SEQ ID NO: 33425 - protein, 9 aa, synthetic construct
GGAGWDTLN

SEQ ID NO: 33426 - protein, 9 aa, synthetic construct
GGAGWDTLQ

SEQ ID NO: 33427 - protein, 9 aa, synthetic construct
GGAGWDLLE

SEQ ID NO: 33428 - protein, 9 aa, synthetic construct
GGAGWDGLY

SEQ ID NO: 33429 - protein, 9 aa, synthetic construct
GGAGVDWLD

SEQ ID NO: 33430 - protein, 9 aa, synthetic construct
GGAGWDFLI

SEQ ID NO: 33431 - protein, 9 aa, synthetic construct
GGAGVDWLE

SEQ ID NO: 33432 - protein, 9 aa, synthetic construct
GGAGVDYAA

SEQ ID NO: 33433 - protein, 9 aa, synthetic construct
GGAGVDYFA

SEQ ID NO: 33434 - protein, 9 aa, synthetic construct
GGAGVDYFD

SEQ ID NO: 33435 - protein, 9 aa, synthetic construct
GGAGVDYFQ

SEQ ID NO: 33436 - protein, 9 aa, synthetic construct
GGAGVDYFV

SEQ ID NO: 33437 - protein, 9 aa, synthetic construct
GGAGVDYIL

SEQ ID NO: 33438 - protein, 9 aa, synthetic construct
GGAGVDYLF

SEQ ID NO: 33439 - protein, 9 aa, synthetic construct
GGAGVDYLL

SEQ ID NO: 33440 - protein, 9 aa, synthetic construct
GGAGVDYLR

SEQ ID NO: 33441 - protein, 9 aa, synthetic construct
GGAGVDYLS

SEQ ID NO: 33442 - protein, 9 aa, synthetic construct
GGAGWDAAD

SEQ ID NO: 33443 - protein, 9 aa, synthetic construct
GGAGWDALF

SEQ ID NO: 33444 - protein, 9 aa, synthetic construct
GGAGWDEFI

SEQ ID NO: 33445 - protein, 9 aa, synthetic construct
GGAGWDEFV

SEQ ID NO: 33446 - protein, 9 aa, synthetic construct
GGAGWDEIY

SEQ ID NO: 33447 - protein, 9 aa, synthetic construct
GGAGWDEVV

SEQ ID NO: 33448 - protein, 9 aa, synthetic construct
GGDGDDHLN

SEQ ID NO: 33449 - protein, 9 aa, synthetic construct
GGDGDDHLV

SEQ ID NO: 33450 - protein, 9 aa, synthetic construct
GGDGIDSLV

SEQ ID NO: 33451 - protein, 9 aa, synthetic construct
GGDGGDVIV

SEQ ID NO: 33452 - protein, 9 aa, synthetic construct
GGDGGDTYM

SEQ ID NO: 33453 - protein, 9 aa, synthetic construct
GGDGGDTYV

SEQ ID NO: 33454 - protein, 9 aa, synthetic construct
GGDGGDTYY

SEQ ID NO: 33455 - protein, 9 aa, synthetic construct
GGDGGDVFA

SEQ ID NO: 33456 - protein, 9 aa, synthetic construct
GGDGGDVIA

SEQ ID NO: 33457 - protein, 9 aa, synthetic construct
GGDGGDVID

SEQ ID NO: 33458 - protein, 9 aa, synthetic construct
GGDGGDVIE

SEQ ID NO: 33459 - protein, 9 aa, synthetic construct
GGDGGDVIR

SEQ ID NO: 33460 - protein, 9 aa, synthetic construct
GGDGGDVIW

SEQ ID NO: 33461 - protein, 9 aa, synthetic construct
GGDGHDHLS

SEQ ID NO: 33462 - protein, 9 aa, synthetic construct
GGDGGDVLD

SEQ ID NO: 33463 - protein, 9 aa, synthetic construct
GGDGGDVLE

SEQ ID NO: 33464 - protein, 9 aa, synthetic construct
GGDGGDVLH

SEQ ID NO: 33465 - protein, 9 aa, synthetic construct
GGDGGDVLI

SEQ ID NO: 33466 - protein, 9 aa, synthetic construct
GGDGGDVLL

SEQ ID NO: 33467 - protein, 9 aa, synthetic construct
GGDGGDVYV

SEQ ID NO: 33468 - protein, 9 aa, synthetic construct
GGDGGDWIE

SEQ ID NO: 33469 - protein, 9 aa, synthetic construct
GGDGGDWIY

SEQ ID NO: 33470 - protein, 9 aa, synthetic construct
GGDGGDTYI

SEQ ID NO: 33471 - protein, 9 aa, synthetic construct
GGDGGDTVH

SEQ ID NO: 33472 - protein, 9 aa, synthetic construct
GGDGGDTMD

SEQ ID NO: 33473 - protein, 9 aa, synthetic construct
GGDGGDTLR

SEQ ID NO: 33474 - protein, 9 aa, synthetic construct
GGDGGDSIE

SEQ ID NO: 33475 - protein, 9 aa, synthetic construct
GGDGGDSIS

SEQ ID NO: 33476 - protein, 9 aa, synthetic construct
GGDGGDSIV

SEQ ID NO: 33477 - protein, 9 aa, synthetic construct
GGDGGDSIY

SEQ ID NO: 33478 - protein, 9 aa, synthetic construct
GGDGGDSLL

SEQ ID NO: 33479 - protein, 9 aa, synthetic construct
GGDGGDSLN

SEQ ID NO: 33480 - protein, 9 aa, synthetic construct
GGDGGDSLS

SEQ ID NO: 33481 - protein, 9 aa, synthetic construct
GGDGGDSVT

SEQ ID NO: 33482 - protein, 9 aa, synthetic construct
GGDGGDTAS

SEQ ID NO: 33483 - protein, 9 aa, synthetic construct
GGDGGDTFN

SEQ ID NO: 33484 - protein, 9 aa, synthetic construct
GGDGGDTFS

SEQ ID NO: 33485 - protein, 9 aa, synthetic construct
GGDGGDTID

SEQ ID NO: 33486 - protein, 9 aa, synthetic construct
GGDGGDTIE

SEQ ID NO: 33487 - protein, 9 aa, synthetic construct
GGDGGDTII

SEQ ID NO: 33488 - protein, 9 aa, synthetic construct
GGDGGDTIL

SEQ ID NO: 33489 - protein, 9 aa, synthetic construct
GGDGGDTIQ

SEQ ID NO: 33490 - protein, 9 aa, synthetic construct
GGDGGDTLE

SEQ ID NO: 33491 - protein, 9 aa, synthetic construct
GGDGGDWLE

SEQ ID NO: 33492 - protein, 9 aa, synthetic construct
GGDGGDWLF

SEQ ID NO: 33493 - protein, 9 aa, synthetic construct
GGDGGDWLI

SEQ ID NO: 33494 - protein, 9 aa, synthetic construct
GGDGHDEIL

SEQ ID NO: 33495 - protein, 9 aa, synthetic construct
GGDGHDEIS

SEQ ID NO: 33496 - protein, 9 aa, synthetic construct
GGDGHDEIV

SEQ ID NO: 33497 - protein, 9 aa, synthetic construct
GGDGHDEIW

SEQ ID NO: 33498 - protein, 9 aa, synthetic construct
GGDGHDEIY

SEQ ID NO: 33499 - protein, 9 aa, synthetic construct
GGDGHDELF

SEQ ID NO: 33500 - protein, 9 aa, synthetic construct
GGDGHDELN

SEQ ID NO: 33501 - protein, 9 aa, synthetic construct
GGDGHDELT

SEQ ID NO: 33502 - protein, 9 aa, synthetic construct
GGDGHDELY

SEQ ID NO: 33503 - protein, 9 aa, synthetic construct
GGDGHDFAS

SEQ ID NO: 33504 - protein, 9 aa, synthetic construct
GGDGHDFIE

SEQ ID NO: 33505 - protein, 9 aa, synthetic construct
GGDGHDFLI

SEQ ID NO: 33506 - protein, 9 aa, synthetic construct
GGDGHDFLW

SEQ ID NO: 33507 - protein, 9 aa, synthetic construct
GGDGHDFLY

SEQ ID NO: 33508 - protein, 9 aa, synthetic construct
GGDGHDFME

SEQ ID NO: 33509 - protein, 9 aa, synthetic construct
GGDGHDFVY

SEQ ID NO: 33510 - protein, 9 aa, synthetic construct
GGDGHDGIK

SEQ ID NO: 33511 - protein, 9 aa, synthetic construct
GGDGHDHIR

SEQ ID NO: 33512 - protein, 9 aa, synthetic construct
GGDGHDEIR

SEQ ID NO: 33513 - protein, 9 aa, synthetic construct
GGDGHDDLY

SEQ ID NO: 33514 - protein, 9 aa, synthetic construct
GGDGGDWLN

SEQ ID NO: 33515 - protein, 9 aa, synthetic construct
GGDGHDDLW

SEQ ID NO: 33516 - protein, 9 aa, synthetic construct
GGDGGDWVR

SEQ ID NO: 33517 - protein, 9 aa, synthetic construct
GGDGGDYFR

SEQ ID NO: 33518 - protein, 9 aa, synthetic construct
GGDGGDYLF

SEQ ID NO: 33519 - protein, 9 aa, synthetic construct
GGDGGDYLG

SEQ ID NO: 33520 - protein, 9 aa, synthetic construct
GGDGGDYLS

SEQ ID NO: 33521 - protein, 9 aa, synthetic construct
GGDGGDYYH

SEQ ID NO: 33522 - protein, 9 aa, synthetic construct
GGDGHDALN

SEQ ID NO: 33523 - protein, 9 aa, synthetic construct
GGDGHDALV

SEQ ID NO: 33524 - protein, 9 aa, synthetic construct
GGDGHDAMA

SEQ ID NO: 33525 - protein, 9 aa, synthetic construct
GGDGHDAVI

SEQ ID NO: 33526 - protein, 9 aa, synthetic construct
GGDGHDDII

SEQ ID NO: 33527 - protein, 9 aa, synthetic construct
GGDGHDDIN

SEQ ID NO: 33528 - protein, 9 aa, synthetic construct
GGDGHDDIY

SEQ ID NO: 33529 - protein, 9 aa, synthetic construct
GGDGHDDLD

SEQ ID NO: 33530 - protein, 9 aa, synthetic construct
GGDGHDDLH

SEQ ID NO: 33531 - protein, 9 aa, synthetic construct
GGDGHDDLR

SEQ ID NO: 33532 - protein, 9 aa, synthetic construct
GGDGHDDLS

SEQ ID NO: 33533 - protein, 9 aa, synthetic construct
GGDGGDSID

SEQ ID NO: 33534 - protein, 9 aa, synthetic construct
GGDGGDRLW

SEQ ID NO: 33535 - protein, 9 aa, synthetic construct
GGDGGDRLT

SEQ ID NO: 33536 - protein, 9 aa, synthetic construct
GGDGFDWLR

SEQ ID NO: 33537 - protein, 9 aa, synthetic construct
GGDGFDYAF

SEQ ID NO: 33538 - protein, 9 aa, synthetic construct
GGDGFDYVD

SEQ ID NO: 33539 - protein, 9 aa, synthetic construct
GGDGFDYVS

SEQ ID NO: 33540 - protein, 9 aa, synthetic construct
GGDGGDAAA

SEQ ID NO: 33541 - protein, 9 aa, synthetic construct
GGDGGDAFQ

SEQ ID NO: 33542 - protein, 9 aa, synthetic construct
GGDGGDALD

SEQ ID NO: 33543 - protein, 9 aa, synthetic construct
GGDGGDALK

SEQ ID NO: 33544 - protein, 9 aa, synthetic construct
GGDGGDALN

SEQ ID NO: 33545 - protein, 9 aa, synthetic construct
GGDGGDALS

SEQ ID NO: 33546 - protein, 9 aa, synthetic construct
GGDGGDCAD

SEQ ID NO: 33547 - protein, 9 aa, synthetic construct
GGDGGDDIH

SEQ ID NO: 33548 - protein, 9 aa, synthetic construct
GGDGGDDIT

SEQ ID NO: 33549 - protein, 9 aa, synthetic construct
GGDGGDDYV

SEQ ID NO: 33550 - protein, 9 aa, synthetic construct
GGDGGDEID

SEQ ID NO: 33551 - protein, 9 aa, synthetic construct
GGDGGDELH

SEQ ID NO: 33552 - protein, 9 aa, synthetic construct
GGDGGDELW

SEQ ID NO: 33553 - protein, 9 aa, synthetic construct
GGDGGDFIN

SEQ ID NO: 33554 - protein, 9 aa, synthetic construct
GGDGFDWVR

SEQ ID NO: 33555 - protein, 9 aa, synthetic construct
GGDGFDVYH

SEQ ID NO: 33556 - protein, 9 aa, synthetic construct
GGDGGDFLQ

SEQ ID NO: 33557 - protein, 9 aa, synthetic construct
GGDGFDVIT

SEQ ID NO: 33558 - protein, 9 aa, synthetic construct
GGDGFDTAT

SEQ ID NO: 33559 - protein, 9 aa, synthetic construct
GGDGFDTFI

SEQ ID NO: 33560 - protein, 9 aa, synthetic construct
GGDGFDTFT

SEQ ID NO: 33561 - protein, 9 aa, synthetic construct
GGDGFDTIA

SEQ ID NO: 33562 - protein, 9 aa, synthetic construct
GGDGFDTIF

SEQ ID NO: 33563 - protein, 9 aa, synthetic construct
GGDGFDTIH

SEQ ID NO: 33564 - protein, 9 aa, synthetic construct
GGDGFDTIS

SEQ ID NO: 33565 - protein, 9 aa, synthetic construct
GGDGFDTLR

SEQ ID NO: 33566 - protein, 9 aa, synthetic construct
GGDGFDTLS

SEQ ID NO: 33567 - protein, 9 aa, synthetic construct
GGDGFDTMV

SEQ ID NO: 33568 - protein, 9 aa, synthetic construct
GGDGFDTYM

SEQ ID NO: 33569 - protein, 9 aa, synthetic construct
GGDGFDTYR

SEQ ID NO: 33570 - protein, 9 aa, synthetic construct
GGDGFDVAA

SEQ ID NO: 33571 - protein, 9 aa, synthetic construct
GGDGFDVAV

SEQ ID NO: 33572 - protein, 9 aa, synthetic construct
GGDGFDVFI

SEQ ID NO: 33573 - protein, 9 aa, synthetic construct
GGDGFDVFV

SEQ ID NO: 33574 - protein, 9 aa, synthetic construct
GGDGFDVIR

SEQ ID NO: 33575 - protein, 9 aa, synthetic construct
GGDGGDFLN

SEQ ID NO: 33576 - protein, 9 aa, synthetic construct
GGDGGDFVY

SEQ ID NO: 33577 - protein, 9 aa, synthetic construct
GGDGGDRLS

SEQ ID NO: 33578 - protein, 9 aa, synthetic construct
GGDGGDMLH

SEQ ID NO: 33579 - protein, 9 aa, synthetic construct
GGDGGDNLE

SEQ ID NO: 33580 - protein, 9 aa, synthetic construct
GGDGGDNLQ

SEQ ID NO: 33581 - protein, 9 aa, synthetic construct
GGDGGDNLY

SEQ ID NO: 33582 - protein, 9 aa, synthetic construct
GGDGGDNVY

SEQ ID NO: 33583 - protein, 9 aa, synthetic construct
GGDGGDQIH

SEQ ID NO: 33584 - protein, 9 aa, synthetic construct
GGDGGDQIS

SEQ ID NO: 33585 - protein, 9 aa, synthetic construct
GGDGGDQLF

SEQ ID NO: 33586 - protein, 9 aa, synthetic construct
GGDGGDQLK

SEQ ID NO: 33587 - protein, 9 aa, synthetic construct
GGDGGDQLL

SEQ ID NO: 33588 - protein, 9 aa, synthetic construct
GGDGGDQLY

SEQ ID NO: 33589 - protein, 9 aa, synthetic construct
GGDGGDQVD

SEQ ID NO: 33590 - protein, 9 aa, synthetic construct
GGDGGDRFF

SEQ ID NO: 33591 - protein, 9 aa, synthetic construct
GGDGGDRFR

SEQ ID NO: 33592 - protein, 9 aa, synthetic construct
GGDGGDRID

SEQ ID NO: 33593 - protein, 9 aa, synthetic construct
GGDGGDRIE

SEQ ID NO: 33594 - protein, 9 aa, synthetic construct
GGDGGDRLA

SEQ ID NO: 33595 - protein, 9 aa, synthetic construct
GGDGGDRLK

SEQ ID NO: 33596 - protein, 9 aa, synthetic construct
GGDGGDMLS

SEQ ID NO: 33597 - protein, 9 aa, synthetic construct
GGDGGDLYI

SEQ ID NO: 33598 - protein, 9 aa, synthetic construct
GGDGGDGAA

SEQ ID NO: 33599 - protein, 9 aa, synthetic construct
GGDGGDLMT

SEQ ID NO: 33600 - protein, 9 aa, synthetic construct
GGDGGDGLE

SEQ ID NO: 33601 - protein, 9 aa, synthetic construct
GGDGGDGLF

SEQ ID NO: 33602 - protein, 9 aa, synthetic construct
GGDGGDGLI

SEQ ID NO: 33603 - protein, 9 aa, synthetic construct
GGDGGDHLY

SEQ ID NO: 33604 - protein, 9 aa, synthetic construct
GGDGGDIIG

SEQ ID NO: 33605 - protein, 9 aa, synthetic construct
GGDGGDILL

SEQ ID NO: 33606 - protein, 9 aa, synthetic construct
GGDGGDILV

SEQ ID NO: 33607 - protein, 9 aa, synthetic construct
GGDGGDIVS

SEQ ID NO: 33608 - protein, 9 aa, synthetic construct
GGDGGDKLI

SEQ ID NO: 33609 - protein, 9 aa, synthetic construct
GGDGGDLIE

SEQ ID NO: 33610 - protein, 9 aa, synthetic construct
GGDGGDLIN

SEQ ID NO: 33611 - protein, 9 aa, synthetic construct
GGDGGDLLI

SEQ ID NO: 33612 - protein, 9 aa, synthetic construct
GGDGGDLLN

SEQ ID NO: 33613 - protein, 9 aa, synthetic construct
GGDGGDLLS

SEQ ID NO: 33614 - protein, 9 aa, synthetic construct
GGDGGDLLV

SEQ ID NO: 33615 - protein, 9 aa, synthetic construct
GGDGGDLMR

SEQ ID NO: 33616 - protein, 9 aa, synthetic construct
GGDGGDLMS

SEQ ID NO: 33617 - protein, 9 aa, synthetic construct
GGDGHDHLQ

SEQ ID NO: 33618 - protein, 9 aa, synthetic construct
GGDGHDHVY

SEQ ID NO: 33619 - protein, 9 aa, synthetic construct
GGDGDDHLX

SEQ ID NO: 33620 - protein, 9 aa, synthetic construct
GGDGIDGLR

SEQ ID NO: 33621 - protein, 9 aa, synthetic construct
GGDGIDEMA

SEQ ID NO: 33622 - protein, 9 aa, synthetic construct
GGDGIDEVD

SEQ ID NO: 33623 - protein, 9 aa, synthetic construct
GGDGIDEVR

SEQ ID NO: 33624 - protein, 9 aa, synthetic construct
GGDGIDFAY

SEQ ID NO: 33625 - protein, 9 aa, synthetic construct
GGDGIDFLA

SEQ ID NO: 33626 - protein, 9 aa, synthetic construct
GGDGIDFVA

SEQ ID NO: 33627 - protein, 9 aa, synthetic construct
GGDGIDFVL

SEQ ID NO: 33628 - protein, 9 aa, synthetic construct
GGDGIDFVV

SEQ ID NO: 33629 - protein, 9 aa, synthetic construct
GGDGIDGLY

SEQ ID NO: 33630 - protein, 9 aa, synthetic construct
GGDGHDIAD

SEQ ID NO: 33631 - protein, 9 aa, synthetic construct
GGDGIDHFV

SEQ ID NO: 33632 - protein, 9 aa, synthetic construct
GGDGIDHLD

SEQ ID NO: 33633 - protein, 9 aa, synthetic construct
GGDGIDHLR

SEQ ID NO: 33634 - protein, 9 aa, synthetic construct
GGDGIDHLY

SEQ ID NO: 33635 - protein, 9 aa, synthetic construct
GGDGIDIAE

SEQ ID NO: 33636 - protein, 9 aa, synthetic construct
GGDGIDIFA

SEQ ID NO: 33637 - protein, 9 aa, synthetic construct
GGDGIDIID

SEQ ID NO: 33638 - protein, 9 aa, synthetic construct
GGDGIDIIV

SEQ ID NO: 33639 - protein, 9 aa, synthetic construct
GGDGIDELQ

SEQ ID NO: 33640 - protein, 9 aa, synthetic construct
GGDGIDELN

SEQ ID NO: 33641 - protein, 9 aa, synthetic construct
GGDGIDELI

SEQ ID NO: 33642 - protein, 9 aa, synthetic construct
GGDGIDELF

SEQ ID NO: 33643 - protein, 9 aa, synthetic construct
GGDGHDYIE

SEQ ID NO: 33644 - protein, 9 aa, synthetic construct
GGDGHDYIS

SEQ ID NO: 33645 - protein, 9 aa, synthetic construct
GGDGHDYLN

SEQ ID NO: 33646 - protein, 9 aa, synthetic construct
GGDGHDYLS

SEQ ID NO: 33647 - protein, 9 aa, synthetic construct
GGDGHDYLY

SEQ ID NO: 33648 - protein, 9 aa, synthetic construct
GGDGHDYVG

SEQ ID NO: 33649 - protein, 9 aa, synthetic construct
GGDGHDYVY

SEQ ID NO: 33650 - protein, 9 aa, synthetic construct
GGDGIDAAA

SEQ ID NO: 33651 - protein, 9 aa, synthetic construct
GGDGIDAAD

SEQ ID NO: 33652 - protein, 9 aa, synthetic construct
GGDGIDAAG

SEQ ID NO: 33653 - protein, 9 aa, synthetic construct
GGDGIDAAY

SEQ ID NO: 33654 - protein, 9 aa, synthetic construct
GGDGIDAIY

SEQ ID NO: 33655 - protein, 9 aa, synthetic construct
GGDGIDALA

SEQ ID NO: 33656 - protein, 9 aa, synthetic construct
GGDGIDALS

SEQ ID NO: 33657 - protein, 9 aa, synthetic construct
GGDGIDAVI

SEQ ID NO: 33658 - protein, 9 aa, synthetic construct
GGDGIDDLY

SEQ ID NO: 33659 - protein, 9 aa, synthetic construct
GGDGIDDVS

SEQ ID NO: 33660 - protein, 9 aa, synthetic construct
GGDGIDILK

SEQ ID NO: 33661 - protein, 9 aa, synthetic construct
GGDGIDILL

SEQ ID NO: 33662 - protein, 9 aa, synthetic construct
GGDGIDILR

SEQ ID NO: 33663 - protein, 9 aa, synthetic construct
GGDGIDQFR

SEQ ID NO: 33664 - protein, 9 aa, synthetic construct
GGDGIDRAD

SEQ ID NO: 33665 - protein, 9 aa, synthetic construct
GGDGIDRAQ

SEQ ID NO: 33666 - protein, 9 aa, synthetic construct
GGDGIDRFA

SEQ ID NO: 33667 - protein, 9 aa, synthetic construct
GGDGIDRIF

SEQ ID NO: 33668 - protein, 9 aa, synthetic construct
GGDGIDRIN

SEQ ID NO: 33669 - protein, 9 aa, synthetic construct
GGDGIDRLA

SEQ ID NO: 33670 - protein, 9 aa, synthetic construct
GGDGIDRLF

SEQ ID NO: 33671 - protein, 9 aa, synthetic construct
GGDGIDRLI

SEQ ID NO: 33672 - protein, 9 aa, synthetic construct
GGDGIDRLQ

SEQ ID NO: 33673 - protein, 9 aa, synthetic construct
GGDGIDRLV

SEQ ID NO: 33674 - protein, 9 aa, synthetic construct
GGDGIDRLY

SEQ ID NO: 33675 - protein, 9 aa, synthetic construct
GGDGIDRMA

SEQ ID NO: 33676 - protein, 9 aa, synthetic construct
GGDGIDRVD

SEQ ID NO: 33677 - protein, 9 aa, synthetic construct
GGDGIDSIY

SEQ ID NO: 33678 - protein, 9 aa, synthetic construct
GGDGIDSLI

SEQ ID NO: 33679 - protein, 9 aa, synthetic construct
GGDGIDSLN

SEQ ID NO: 33680 - protein, 9 aa, synthetic construct
GGDGIDSLS

SEQ ID NO: 33681 - protein, 9 aa, synthetic construct
GGDGIDQLS

SEQ ID NO: 33682 - protein, 9 aa, synthetic construct
GGDGIDNVW

SEQ ID NO: 33683 - protein, 9 aa, synthetic construct
GGDGIDILS

SEQ ID NO: 33684 - protein, 9 aa, synthetic construct
GGDGIDNVA

SEQ ID NO: 33685 - protein, 9 aa, synthetic construct
GGDGIDILY

SEQ ID NO: 33686 - protein, 9 aa, synthetic construct
GGDGIDIML

SEQ ID NO: 33687 - protein, 9 aa, synthetic construct
GGDGIDIMY

SEQ ID NO: 33688 - protein, 9 aa, synthetic construct
GGDGIDIVL

SEQ ID NO: 33689 - protein, 9 aa, synthetic construct
GGDGIDIVS

SEQ ID NO: 33690 - protein, 9 aa, synthetic construct
GGDGIDLIL

SEQ ID NO: 33691 - protein, 9 aa, synthetic construct
GGDGIDLLI

SEQ ID NO: 33692 - protein, 9 aa, synthetic construct
GGDGIDLLN

SEQ ID NO: 33693 - protein, 9 aa, synthetic construct
GGDGIDLMV

SEQ ID NO: 33694 - protein, 9 aa, synthetic construct
GGDGIDLVL

SEQ ID NO: 33695 - protein, 9 aa, synthetic construct
GGDGIDLVS

SEQ ID NO: 33696 - protein, 9 aa, synthetic construct
GGDGIDMIS

SEQ ID NO: 33697 - protein, 9 aa, synthetic construct
GGDGIDMLF

SEQ ID NO: 33698 - protein, 9 aa, synthetic construct
GGDGIDMLV

SEQ ID NO: 33699 - protein, 9 aa, synthetic construct
GGDGIDMVS

SEQ ID NO: 33700 - protein, 9 aa, synthetic construct
GGDGIDNID

SEQ ID NO: 33701 - protein, 9 aa, synthetic construct
GGDGIDNIN

SEQ ID NO: 33702 - protein, 9 aa, synthetic construct
GGDGHDYAD

SEQ ID NO: 33703 - protein, 9 aa, synthetic construct
GGDGHDWLH

SEQ ID NO: 33704 - protein, 9 aa, synthetic construct
GGDGHDWLF

SEQ ID NO: 33705 - protein, 9 aa, synthetic construct
GGDGHDLMY

SEQ ID NO: 33706 - protein, 9 aa, synthetic construct
GGDGHDLVQ

SEQ ID NO: 33707 - protein, 9 aa, synthetic construct
GGDGHDMLI

SEQ ID NO: 33708 - protein, 9 aa, synthetic construct
GGDGHDMLR

SEQ ID NO: 33709 - protein, 9 aa, synthetic construct
GGDGHDNIE

SEQ ID NO: 33710 - protein, 9 aa, synthetic construct
GGDGHDNIG

SEQ ID NO: 33711 - protein, 9 aa, synthetic construct
GGDGHDNIS

SEQ ID NO: 33712 - protein, 9 aa, synthetic construct
GGDGHDNLI

SEQ ID NO: 33713 - protein, 9 aa, synthetic construct
GGDGHDNLK

SEQ ID NO: 33714 - protein, 9 aa, synthetic construct
GGDGHDNMA

SEQ ID NO: 33715 - protein, 9 aa, synthetic construct
GGDGHDNYN

SEQ ID NO: 33716 - protein, 9 aa, synthetic construct
GGDGHDQAI

SEQ ID NO: 33717 - protein, 9 aa, synthetic construct
GGDGHDQFV

SEQ ID NO: 33718 - protein, 9 aa, synthetic construct
GGDGHDQIN

SEQ ID NO: 33719 - protein, 9 aa, synthetic construct
GGDGHDQLK

SEQ ID NO: 33720 - protein, 9 aa, synthetic construct
GGDGHDQLR

SEQ ID NO: 33721 - protein, 9 aa, synthetic construct
GGDGHDQLY

SEQ ID NO: 33722 - protein, 9 aa, synthetic construct
GGDGHDQMY

SEQ ID NO: 33723 - protein, 9 aa, synthetic construct
GGDGHDLVN

SEQ ID NO: 33724 - protein, 9 aa, synthetic construct
GGDGHDLLR

SEQ ID NO: 33725 - protein, 9 aa, synthetic construct
GGDGHDRFV

SEQ ID NO: 33726 - protein, 9 aa, synthetic construct
GGDGHDLLN

SEQ ID NO: 33727 - protein, 9 aa, synthetic construct
GGDGHDIIH

SEQ ID NO: 33728 - protein, 9 aa, synthetic construct
GGDGHDIIK

SEQ ID NO: 33729 - protein, 9 aa, synthetic construct
GGDGHDIIL

SEQ ID NO: 33730 - protein, 9 aa, synthetic construct
GGDGHDILF

SEQ ID NO: 33731 - protein, 9 aa, synthetic construct
GGDGHDILH

SEQ ID NO: 33732 - protein, 9 aa, synthetic construct
GGDGHDILS

SEQ ID NO: 33733 - protein, 9 aa, synthetic construct
GGDGHDIMI

SEQ ID NO: 33734 - protein, 9 aa, synthetic construct
GGDGHDIYV

SEQ ID NO: 33735 - protein, 9 aa, synthetic construct
GGDGHDKIV

SEQ ID NO: 33736 - protein, 9 aa, synthetic construct
GGDGHDKIY

SEQ ID NO: 33737 - protein, 9 aa, synthetic construct
GGDGHDKLV

SEQ ID NO: 33738 - protein, 9 aa, synthetic construct
GGDGHDKVN

SEQ ID NO: 33739 - protein, 9 aa, synthetic construct
GGDGHDLAY

SEQ ID NO: 33740 - protein, 9 aa, synthetic construct
GGDGHDLFL

SEQ ID NO: 33741 - protein, 9 aa, synthetic construct
GGDGHDLIA

SEQ ID NO: 33742 - protein, 9 aa, synthetic construct
GGDGHDLID

SEQ ID NO: 33743 - protein, 9 aa, synthetic construct
GGDGHDLLG

SEQ ID NO: 33744 - protein, 9 aa, synthetic construct
GGDGHDQVF

SEQ ID NO: 33745 - protein, 9 aa, synthetic construct
GGDGHDRFY

SEQ ID NO: 33746 - protein, 9 aa, synthetic construct
GGDGHDWLE

SEQ ID NO: 33747 - protein, 9 aa, synthetic construct
GGDGHDTLH

SEQ ID NO: 33748 - protein, 9 aa, synthetic construct
GGDGHDTMS

SEQ ID NO: 33749 - protein, 9 aa, synthetic construct
GGDGHDTMY

SEQ ID NO: 33750 - protein, 9 aa, synthetic construct
GGDGHDTVD

SEQ ID NO: 33751 - protein, 9 aa, synthetic construct
GGDGHDTVL

SEQ ID NO: 33752 - protein, 9 aa, synthetic construct
GGDGHDTVR

SEQ ID NO: 33753 - protein, 9 aa, synthetic construct
GGDGHDVFA

SEQ ID NO: 33754 - protein, 9 aa, synthetic construct
GGDGHDVFS

SEQ ID NO: 33755 - protein, 9 aa, synthetic construct
GGDGHDVFV

SEQ ID NO: 33756 - protein, 9 aa, synthetic construct
GGDGHDVID

SEQ ID NO: 33757 - protein, 9 aa, synthetic construct
GGDGHDVIE

SEQ ID NO: 33758 - protein, 9 aa, synthetic construct
GGDGHDVIR

SEQ ID NO: 33759 - protein, 9 aa, synthetic construct
GGDGHDVLM

SEQ ID NO: 33760 - protein, 9 aa, synthetic construct
GGDGHDVLW

SEQ ID NO: 33761 - protein, 9 aa, synthetic construct
GGDGHDVVN

SEQ ID NO: 33762 - protein, 9 aa, synthetic construct
GGDGHDVYA

SEQ ID NO: 33763 - protein, 9 aa, synthetic construct
GGDGHDWID

SEQ ID NO: 33764 - protein, 9 aa, synthetic construct
GGDGHDWLD

SEQ ID NO: 33765 - protein, 9 aa, synthetic construct
GGDGHDTMI

SEQ ID NO: 33766 - protein, 9 aa, synthetic construct
GGDGHDTIT

SEQ ID NO: 33767 - protein, 9 aa, synthetic construct
GGDGHDRID

SEQ ID NO: 33768 - protein, 9 aa, synthetic construct
GGDGHDTIE

SEQ ID NO: 33769 - protein, 9 aa, synthetic construct
GGDGHDRIW

SEQ ID NO: 33770 - protein, 9 aa, synthetic construct
GGDGHDRIY

SEQ ID NO: 33771 - protein, 9 aa, synthetic construct
GGDGHDRLG

SEQ ID NO: 33772 - protein, 9 aa, synthetic construct
GGDGHDRMF

SEQ ID NO: 33773 - protein, 9 aa, synthetic construct
GGDGHDSIE

SEQ ID NO: 33774 - protein, 9 aa, synthetic construct
GGDGHDSIH

SEQ ID NO: 33775 - protein, 9 aa, synthetic construct
GGDGHDSIV

SEQ ID NO: 33776 - protein, 9 aa, synthetic construct
GGDGHDSIY

SEQ ID NO: 33777 - protein, 9 aa, synthetic construct
GGDGHDSLN

SEQ ID NO: 33778 - protein, 9 aa, synthetic construct
GGDGHDSLR

SEQ ID NO: 33779 - protein, 9 aa, synthetic construct
GGDGHDSME

SEQ ID NO: 33780 - protein, 9 aa, synthetic construct
GGDGHDSVS

SEQ ID NO: 33781 - protein, 9 aa, synthetic construct
GGDGHDSVT

SEQ ID NO: 33782 - protein, 9 aa, synthetic construct
GGDGHDTAS

SEQ ID NO: 33783 - protein, 9 aa, synthetic construct
GGDGHDTFM

SEQ ID NO: 33784 - protein, 9 aa, synthetic construct
GGDGHDTFN

SEQ ID NO: 33785 - protein, 9 aa, synthetic construct
GGDGHDTFR

SEQ ID NO: 33786 - protein, 9 aa, synthetic construct
GGDGFDTAI

SEQ ID NO: 33787 - protein, 9 aa, synthetic construct
GGDGFDTAH

SEQ ID NO: 33788 - protein, 9 aa, synthetic construct
GGDGFDTAF

SEQ ID NO: 33789 - protein, 9 aa, synthetic construct
GGDGDDSVV

SEQ ID NO: 33790 - protein, 9 aa, synthetic construct
GGDGDDRYY

SEQ ID NO: 33791 - protein, 9 aa, synthetic construct
GGDGDDSFT

SEQ ID NO: 33792 - protein, 9 aa, synthetic construct
GGDGDDSIW

SEQ ID NO: 33793 - protein, 9 aa, synthetic construct
GGDGDDSMF

SEQ ID NO: 33794 - protein, 9 aa, synthetic construct
GGDGDDSMG

SEQ ID NO: 33795 - protein, 9 aa, synthetic construct
GGDGDDSMH

SEQ ID NO: 33796 - protein, 9 aa, synthetic construct
GGDGDDSMI

SEQ ID NO: 33797 - protein, 9 aa, synthetic construct
GGDGDDSVQ

SEQ ID NO: 33798 - protein, 9 aa, synthetic construct
GGDGDDSYD

SEQ ID NO: 33799 - protein, 9 aa, synthetic construct
GGDGFDTAA

SEQ ID NO: 33800 - protein, 9 aa, synthetic construct
GGDGDDSYS

SEQ ID NO: 33801 - protein, 9 aa, synthetic construct
GGDGDDTAH

SEQ ID NO: 33802 - protein, 9 aa, synthetic construct
GGDGDDTAL

SEQ ID NO: 33803 - protein, 9 aa, synthetic construct
GGDGDDTFD

SEQ ID NO: 33804 - protein, 9 aa, synthetic construct
GGDGDDTFQ

SEQ ID NO: 33805 - protein, 9 aa, synthetic construct
GGDGDDTFS

SEQ ID NO: 33806 - protein, 9 aa, synthetic construct
GGDGDDTMG

SEQ ID NO: 33807 - protein, 9 aa, synthetic construct
GGDGDDTMH

SEQ ID NO: 33808 - protein, 9 aa, synthetic construct
GGDGDDRYV

SEQ ID NO: 33809 - protein, 9 aa, synthetic construct
GGDGDDRVV

SEQ ID NO: 33810 - protein, 9 aa, synthetic construct
GGDGDDRVR

SEQ ID NO: 33811 - protein, 9 aa, synthetic construct
GGDGDDRVI

SEQ ID NO: 33812 - protein, 9 aa, synthetic construct
GGDGDDQVI

SEQ ID NO: 33813 - protein, 9 aa, synthetic construct
GGDGDDQVK

SEQ ID NO: 33814 - protein, 9 aa, synthetic construct
GGDGDDQVT

SEQ ID NO: 33815 - protein, 9 aa, synthetic construct
GGDGDDQVV

SEQ ID NO: 33816 - protein, 9 aa, synthetic construct
GGDGDDRAD

SEQ ID NO: 33817 - protein, 9 aa, synthetic construct
GGDGDDRFF

SEQ ID NO: 33818 - protein, 9 aa, synthetic construct
GGDGDDRFL

SEQ ID NO: 33819 - protein, 9 aa, synthetic construct
GGDGDDRFN

SEQ ID NO: 33820 - protein, 9 aa, synthetic construct
GGDGDDRFT

SEQ ID NO: 33821 - protein, 9 aa, synthetic construct
GGDGDDRIQ

SEQ ID NO: 33822 - protein, 9 aa, synthetic construct
GGDGDDRIR

SEQ ID NO: 33823 - protein, 9 aa, synthetic construct
GGDGDDRLK

SEQ ID NO: 33824 - protein, 9 aa, synthetic construct
GGDGDDRMA

SEQ ID NO: 33825 - protein, 9 aa, synthetic construct
GGDGDDRMF

SEQ ID NO: 33826 - protein, 9 aa, synthetic construct
GGDGDDRMG

SEQ ID NO: 33827 - protein, 9 aa, synthetic construct
GGDGDDRVG

SEQ ID NO: 33828 - protein, 9 aa, synthetic construct
GGDGDDRVH

SEQ ID NO: 33829 - protein, 9 aa, synthetic construct
GGDGDDTML

SEQ ID NO: 33830 - protein, 9 aa, synthetic construct
GGDGDDTMQ

SEQ ID NO: 33831 - protein, 9 aa, synthetic construct
GGDGDDTMR

SEQ ID NO: 33832 - protein, 9 aa, synthetic construct
GGDGDDWLL

SEQ ID NO: 33833 - protein, 9 aa, synthetic construct
GGDGDDWLV

SEQ ID NO: 33834 - protein, 9 aa, synthetic construct
GGDGDDWMN

SEQ ID NO: 33835 - protein, 9 aa, synthetic construct
GGDGDDWMS

SEQ ID NO: 33836 - protein, 9 aa, synthetic construct
GGDGDDWVH

SEQ ID NO: 33837 - protein, 9 aa, synthetic construct
GGDGDDWVR

SEQ ID NO: 33838 - protein, 9 aa, synthetic construct
GGDGDDYAR

SEQ ID NO: 33839 - protein, 9 aa, synthetic construct
GGDGDDYFD

SEQ ID NO: 33840 - protein, 9 aa, synthetic construct
GGDGDDYFY

SEQ ID NO: 33841 - protein, 9 aa, synthetic construct
GGDGDDYIF

SEQ ID NO: 33842 - protein, 9 aa, synthetic construct
GGDGDDYII

SEQ ID NO: 33843 - protein, 9 aa, synthetic construct
GGDGDDYIQ

SEQ ID NO: 33844 - protein, 9 aa, synthetic construct
GGDGDDYIW

SEQ ID NO: 33845 - protein, 9 aa, synthetic construct
GGDGDDYLK

SEQ ID NO: 33846 - protein, 9 aa, synthetic construct
GGDGDDYLQ

SEQ ID NO: 33847 - protein, 9 aa, synthetic construct
GGDGDDYMS

SEQ ID NO: 33848 - protein, 9 aa, synthetic construct
GGDGDDYVA

SEQ ID NO: 33849 - protein, 9 aa, synthetic construct
GGDGDDYVL

SEQ ID NO: 33850 - protein, 9 aa, synthetic construct
GGDGDDWLQ

SEQ ID NO: 33851 - protein, 9 aa, synthetic construct
GGDGDDWIT

SEQ ID NO: 33852 - protein, 9 aa, synthetic construct
GGDGDDTVK

SEQ ID NO: 33853 - protein, 9 aa, synthetic construct
GGDGDDWIL

SEQ ID NO: 33854 - protein, 9 aa, synthetic construct
GGDGDDTVQ

SEQ ID NO: 33855 - protein, 9 aa, synthetic construct
GGDGDDTYN

SEQ ID NO: 33856 - protein, 9 aa, synthetic construct
GGDGDDTYR

SEQ ID NO: 33857 - protein, 9 aa, synthetic construct
GGDGDDVAA

SEQ ID NO: 33858 - protein, 9 aa, synthetic construct
GGDGDDVFN

SEQ ID NO: 33859 - protein, 9 aa, synthetic construct
GGDGDDVIK

SEQ ID NO: 33860 - protein, 9 aa, synthetic construct
GGDGDDVMK

SEQ ID NO: 33861 - protein, 9 aa, synthetic construct
GGDGDDVML

SEQ ID NO: 33862 - protein, 9 aa, synthetic construct
GGDGDDVMN

SEQ ID NO: 33863 - protein, 9 aa, synthetic construct
GGDGDDVMR

SEQ ID NO: 33864 - protein, 9 aa, synthetic construct
GGDGDDVMS

SEQ ID NO: 33865 - protein, 9 aa, synthetic construct
GGDGDDVVM

SEQ ID NO: 33866 - protein, 9 aa, synthetic construct
GGDGDDVVV

SEQ ID NO: 33867 - protein, 9 aa, synthetic construct
GGDGDDVYW

SEQ ID NO: 33868 - protein, 9 aa, synthetic construct
GGDGDDWFV

SEQ ID NO: 33869 - protein, 9 aa, synthetic construct
GGDGDDWIF

SEQ ID NO: 33870 - protein, 9 aa, synthetic construct
GGDGDDWIH

SEQ ID NO: 33871 - protein, 9 aa, synthetic construct
GGDGDDQVA

SEQ ID NO: 33872 - protein, 9 aa, synthetic construct
GGDGDDQLN

SEQ ID NO: 33873 - protein, 9 aa, synthetic construct
GGDGDDQLM

SEQ ID NO: 33874 - protein, 9 aa, synthetic construct
GGDGDDIVE

SEQ ID NO: 33875 - protein, 9 aa, synthetic construct
GGDGDDIVH

SEQ ID NO: 33876 - protein, 9 aa, synthetic construct
GGDGDDIVK

SEQ ID NO: 33877 - protein, 9 aa, synthetic construct
GGDGDDIVM

SEQ ID NO: 33878 - protein, 9 aa, synthetic construct
GGDGDDIYH

SEQ ID NO: 33879 - protein, 9 aa, synthetic construct
GGDGDDIYN

SEQ ID NO: 33880 - protein, 9 aa, synthetic construct
GGDGDDIYS

SEQ ID NO: 33881 - protein, 9 aa, synthetic construct
GGDGDDIYT

SEQ ID NO: 33882 - protein, 9 aa, synthetic construct
GGDGDDKII

SEQ ID NO: 33883 - protein, 9 aa, synthetic construct
GGDGDDKLA

SEQ ID NO: 33884 - protein, 9 aa, synthetic construct
GGDGDDKLE

SEQ ID NO: 33885 - protein, 9 aa, synthetic construct
GGDGDDKLH

SEQ ID NO: 33886 - protein, 9 aa, synthetic construct
GGDGDDKLQ

SEQ ID NO: 33887 - protein, 9 aa, synthetic construct
GGDGDDKMF

SEQ ID NO: 33888 - protein, 9 aa, synthetic construct
GGDGDDKVA

SEQ ID NO: 33889 - protein, 9 aa, synthetic construct
GGDGDDKVE

SEQ ID NO: 33890 - protein, 9 aa, synthetic construct
GGDGDDKVW

SEQ ID NO: 33891 - protein, 9 aa, synthetic construct
GGDGDDLAM

SEQ ID NO: 33892 - protein, 9 aa, synthetic construct
GGDGDDIVG

SEQ ID NO: 33893 - protein, 9 aa, synthetic construct
GGDGDDIMY

SEQ ID NO: 33894 - protein, 9 aa, synthetic construct
GGDGDDLFF

SEQ ID NO: 33895 - protein, 9 aa, synthetic construct
GGDGDDIMV

SEQ ID NO: 33896 - protein, 9 aa, synthetic construct
GGDGDDHVA

SEQ ID NO: 33897 - protein, 9 aa, synthetic construct
GGDGDDHVH

SEQ ID NO: 33898 - protein, 9 aa, synthetic construct
GGDGDDIAD

SEQ ID NO: 33899 - protein, 9 aa, synthetic construct
GGDGDDIAT

SEQ ID NO: 33900 - protein, 9 aa, synthetic construct
GGDGDDIAV

SEQ ID NO: 33901 - protein, 9 aa, synthetic construct
GGDGDDIFA

SEQ ID NO: 33902 - protein, 9 aa, synthetic construct
GGDGDDIFS

SEQ ID NO: 33903 - protein, 9 aa, synthetic construct
GGDGDDIFW

SEQ ID NO: 33904 - protein, 9 aa, synthetic construct
GGDGDDIIQ

SEQ ID NO: 33905 - protein, 9 aa, synthetic construct
GGDGDDILG

SEQ ID NO: 33906 - protein, 9 aa, synthetic construct
GGDGDDILW

SEQ ID NO: 33907 - protein, 9 aa, synthetic construct
GGDGDDIMI

SEQ ID NO: 33908 - protein, 9 aa, synthetic construct
GGDGDDIMK

SEQ ID NO: 33909 - protein, 9 aa, synthetic construct
GGDGDDIML

SEQ ID NO: 33910 - protein, 9 aa, synthetic construct
GGDGDDIMR

SEQ ID NO: 33911 - protein, 9 aa, synthetic construct
GGDGDDIMS

SEQ ID NO: 33912 - protein, 9 aa, synthetic construct
GGDGDDIMT

SEQ ID NO: 33913 - protein, 9 aa, synthetic construct
GGDGDDLFD

SEQ ID NO: 33914 - protein, 9 aa, synthetic construct
GGDGDDLMH

SEQ ID NO: 33915 - protein, 9 aa, synthetic construct
GGDGDDQLK

SEQ ID NO: 33916 - protein, 9 aa, synthetic construct
GGDGDDMVF

SEQ ID NO: 33917 - protein, 9 aa, synthetic construct
GGDGDDNIG

SEQ ID NO: 33918 - protein, 9 aa, synthetic construct
GGDGDDNIT

SEQ ID NO: 33919 - protein, 9 aa, synthetic construct
GGDGDDNIW

SEQ ID NO: 33920 - protein, 9 aa, synthetic construct
GGDGDDNLF

SEQ ID NO: 33921 - protein, 9 aa, synthetic construct
GGDGDDNLH

SEQ ID NO: 33922 - protein, 9 aa, synthetic construct
GGDGDDNMA

SEQ ID NO: 33923 - protein, 9 aa, synthetic construct
GGDGDDNMG

SEQ ID NO: 33924 - protein, 9 aa, synthetic construct
GGDGDDNMI

SEQ ID NO: 33925 - protein, 9 aa, synthetic construct
GGDGDDNMM

SEQ ID NO: 33926 - protein, 9 aa, synthetic construct
GGDGDDNVD

SEQ ID NO: 33927 - protein, 9 aa, synthetic construct
GGDGDDNVS

SEQ ID NO: 33928 - protein, 9 aa, synthetic construct
GGDGDDQAW

SEQ ID NO: 33929 - protein, 9 aa, synthetic construct
GGDGDDQFL

SEQ ID NO: 33930 - protein, 9 aa, synthetic construct
GGDGDDQIC

SEQ ID NO: 33931 - protein, 9 aa, synthetic construct
GGDGDDQIG

SEQ ID NO: 33932 - protein, 9 aa, synthetic construct
GGDGDDQIH

SEQ ID NO: 33933 - protein, 9 aa, synthetic construct
GGDGDDQIY

SEQ ID NO: 33934 - protein, 9 aa, synthetic construct
GGDGDDNIF

SEQ ID NO: 33935 - protein, 9 aa, synthetic construct
GGDGDDMMF

SEQ ID NO: 33936 - protein, 9 aa, synthetic construct
GGDGDDLMI

SEQ ID NO: 33937 - protein, 9 aa, synthetic construct
GGDGDDMLW

SEQ ID NO: 33938 - protein, 9 aa, synthetic construct
GGDGDDLML

SEQ ID NO: 33939 - protein, 9 aa, synthetic construct
GGDGDDLMV

SEQ ID NO: 33940 - protein, 9 aa, synthetic construct
GGDGDDLMW

SEQ ID NO: 33941 - protein, 9 aa, synthetic construct
GGDGDDLVE

SEQ ID NO: 33942 - protein, 9 aa, synthetic construct
GGDGDDLVG

SEQ ID NO: 33943 - protein, 9 aa, synthetic construct
GGDGDDLVI

SEQ ID NO: 33944 - protein, 9 aa, synthetic construct
GGDGDDLYF

SEQ ID NO: 33945 - protein, 9 aa, synthetic construct
GGDGDDLYR

SEQ ID NO: 33946 - protein, 9 aa, synthetic construct
GGDGDDMAD

SEQ ID NO: 33947 - protein, 9 aa, synthetic construct
GGDGDDMAT

SEQ ID NO: 33948 - protein, 9 aa, synthetic construct
GGDGDDMFW

SEQ ID NO: 33949 - protein, 9 aa, synthetic construct
GGDGDDMIN

SEQ ID NO: 33950 - protein, 9 aa, synthetic construct
GGDGDDMLC

SEQ ID NO: 33951 - protein, 9 aa, synthetic construct
GGDGDDMLH

SEQ ID NO: 33952 - protein, 9 aa, synthetic construct
GGDGDDMLK

SEQ ID NO: 33953 - protein, 9 aa, synthetic construct
GGDGDDMLR

SEQ ID NO: 33954 - protein, 9 aa, synthetic construct
GGDGDDMLS

SEQ ID NO: 33955 - protein, 9 aa, synthetic construct
GGDGEDAFH

SEQ ID NO: 33956 - protein, 9 aa, synthetic construct
GGDGEDAIS

SEQ ID NO: 33957 - protein, 9 aa, synthetic construct
GGDGEDDID

SEQ ID NO: 33958 - protein, 9 aa, synthetic construct
GGDGEDYLA

SEQ ID NO: 33959 - protein, 9 aa, synthetic construct
GGDGEDYLS

SEQ ID NO: 33960 - protein, 9 aa, synthetic construct
GGDGFDALY

SEQ ID NO: 33961 - protein, 9 aa, synthetic construct
GGDGFDAMN

SEQ ID NO: 33962 - protein, 9 aa, synthetic construct
GGDGFDCMI

SEQ ID NO: 33963 - protein, 9 aa, synthetic construct
GGDGFDDIE

SEQ ID NO: 33964 - protein, 9 aa, synthetic construct
GGDGFDDLK

SEQ ID NO: 33965 - protein, 9 aa, synthetic construct
GGDGFDEAS

SEQ ID NO: 33966 - protein, 9 aa, synthetic construct
GGDGFDEVR

SEQ ID NO: 33967 - protein, 9 aa, synthetic construct
GGDGFDFAI

SEQ ID NO: 33968 - protein, 9 aa, synthetic construct
GGDGFDFIE

SEQ ID NO: 33969 - protein, 9 aa, synthetic construct
GGDGFDFIF

SEQ ID NO: 33970 - protein, 9 aa, synthetic construct
GGDGFDFLI

SEQ ID NO: 33971 - protein, 9 aa, synthetic construct
GGDGFDFMT

SEQ ID NO: 33972 - protein, 9 aa, synthetic construct
GGDGFDHLR

SEQ ID NO: 33973 - protein, 9 aa, synthetic construct
GGDGFDIAI

SEQ ID NO: 33974 - protein, 9 aa, synthetic construct
GGDGFDIAQ

SEQ ID NO: 33975 - protein, 9 aa, synthetic construct
GGDGFDIID

SEQ ID NO: 33976 - protein, 9 aa, synthetic construct
GGDGEDYLE

SEQ ID NO: 33977 - protein, 9 aa, synthetic construct
GGDGEDYID

SEQ ID NO: 33978 - protein, 9 aa, synthetic construct
GGDGFDILD

SEQ ID NO: 33979 - protein, 9 aa, synthetic construct
GGDGEDWLS

SEQ ID NO: 33980 - protein, 9 aa, synthetic construct
GGDGEDVIH

SEQ ID NO: 33981 - protein, 9 aa, synthetic construct
GGDGEDVIK

SEQ ID NO: 33982 - protein, 9 aa, synthetic construct
GGDGEDVIV

SEQ ID NO: 33983 - protein, 9 aa, synthetic construct
GGDGEDVIY

SEQ ID NO: 33984 - protein, 9 aa, synthetic construct
GGDGEDVLA

SEQ ID NO: 33985 - protein, 9 aa, synthetic construct
GGDGEDVLE

SEQ ID NO: 33986 - protein, 9 aa, synthetic construct
GGDGEDVLG

SEQ ID NO: 33987 - protein, 9 aa, synthetic construct
GGDGEDVLK

SEQ ID NO: 33988 - protein, 9 aa, synthetic construct
GGDGEDVLL

SEQ ID NO: 33989 - protein, 9 aa, synthetic construct
GGDGEDVLQ

SEQ ID NO: 33990 - protein, 9 aa, synthetic construct
GGDGEDVMA

SEQ ID NO: 33991 - protein, 9 aa, synthetic construct
GGDGEDVMI

SEQ ID NO: 33992 - protein, 9 aa, synthetic construct
GGDGEDVMY

SEQ ID NO: 33993 - protein, 9 aa, synthetic construct
GGDGEDVVD

SEQ ID NO: 33994 - protein, 9 aa, synthetic construct
GGDGEDVVL

SEQ ID NO: 33995 - protein, 9 aa, synthetic construct
GGDGEDVYL

SEQ ID NO: 33996 - protein, 9 aa, synthetic construct
GGDGEDWIG

SEQ ID NO: 33997 - protein, 9 aa, synthetic construct
GGDGFDIIE

SEQ ID NO: 33998 - protein, 9 aa, synthetic construct
GGDGFDILR

SEQ ID NO: 33999 - protein, 9 aa, synthetic construct
GGDGEDVAE

SEQ ID NO: 34000 - protein, 9 aa, synthetic construct
GGDGFDNLD

SEQ ID NO: 34001 - protein, 9 aa, synthetic construct
GGDGFDQII

SEQ ID NO: 34002 - protein, 9 aa, synthetic construct
GGDGFDQLH

SEQ ID NO: 34003 - protein, 9 aa, synthetic construct
GGDGFDQLK

SEQ ID NO: 34004 - protein, 9 aa, synthetic construct
GGDGFDQLN

SEQ ID NO: 34005 - protein, 9 aa, synthetic construct
GGDGFDQLT

SEQ ID NO: 34006 - protein, 9 aa, synthetic construct
GGDGFDQMS

SEQ ID NO: 34007 - protein, 9 aa, synthetic construct
GGDGFDRAY

SEQ ID NO: 34008 - protein, 9 aa, synthetic construct
GGDGFDRFE

SEQ ID NO: 34009 - protein, 9 aa, synthetic construct
GGDGFDRFL

SEQ ID NO: 34010 - protein, 9 aa, synthetic construct
GGDGFDRIE

SEQ ID NO: 34011 - protein, 9 aa, synthetic construct
GGDGFDRIG

SEQ ID NO: 34012 - protein, 9 aa, synthetic construct
GGDGFDRIL

SEQ ID NO: 34013 - protein, 9 aa, synthetic construct
GGDGFDRIQ

SEQ ID NO: 34014 - protein, 9 aa, synthetic construct
GGDGFDRLH

SEQ ID NO: 34015 - protein, 9 aa, synthetic construct
GGDGFDRLS

SEQ ID NO: 34016 - protein, 9 aa, synthetic construct
GGDGFDRLV

SEQ ID NO: 34017 - protein, 9 aa, synthetic construct
GGDGFDSAD

SEQ ID NO: 34018 - protein, 9 aa, synthetic construct
GGDGFDQIA

SEQ ID NO: 34019 - protein, 9 aa, synthetic construct
GGDGFDMVS

SEQ ID NO: 34020 - protein, 9 aa, synthetic construct
GGDGFDILT

SEQ ID NO: 34021 - protein, 9 aa, synthetic construct
GGDGFDMLI

SEQ ID NO: 34022 - protein, 9 aa, synthetic construct
GGDGFDKAQ

SEQ ID NO: 34023 - protein, 9 aa, synthetic construct
GGDGFDKLF

SEQ ID NO: 34024 - protein, 9 aa, synthetic construct
GGDGFDKLL

SEQ ID NO: 34025 - protein, 9 aa, synthetic construct
GGDGFDLAH

SEQ ID NO: 34026 - protein, 9 aa, synthetic construct
GGDGFDLIA

SEQ ID NO: 34027 - protein, 9 aa, synthetic construct
GGDGFDLLA

SEQ ID NO: 34028 - protein, 9 aa, synthetic construct
GGDGFDLLE

SEQ ID NO: 34029 - protein, 9 aa, synthetic construct
GGDGFDLLF

SEQ ID NO: 34030 - protein, 9 aa, synthetic construct
GGDGFDLLL

SEQ ID NO: 34031 - protein, 9 aa, synthetic construct
GGDGFDLLM

SEQ ID NO: 34032 - protein, 9 aa, synthetic construct
GGDGFDLLQ

SEQ ID NO: 34033 - protein, 9 aa, synthetic construct
GGDGFDLLT

SEQ ID NO: 34034 - protein, 9 aa, synthetic construct
GGDGFDLVN

SEQ ID NO: 34035 - protein, 9 aa, synthetic construct
GGDGFDLVR

SEQ ID NO: 34036 - protein, 9 aa, synthetic construct
GGDGFDMAS

SEQ ID NO: 34037 - protein, 9 aa, synthetic construct
GGDGFDMIK

SEQ ID NO: 34038 - protein, 9 aa, synthetic construct
GGDGFDMIS

SEQ ID NO: 34039 - protein, 9 aa, synthetic construct
GGDGEDVID

SEQ ID NO: 34040 - protein, 9 aa, synthetic construct
GGDGEDTVS

SEQ ID NO: 34041 - protein, 9 aa, synthetic construct
GGDGEDDLA

SEQ ID NO: 34042 - protein, 9 aa, synthetic construct
GGDGEDIIV

SEQ ID NO: 34043 - protein, 9 aa, synthetic construct
GGDGEDIMY

SEQ ID NO: 34044 - protein, 9 aa, synthetic construct
GGDGEDIVL

SEQ ID NO: 34045 - protein, 9 aa, synthetic construct
GGDGEDKLF

SEQ ID NO: 34046 - protein, 9 aa, synthetic construct
GGDGEDLIA

SEQ ID NO: 34047 - protein, 9 aa, synthetic construct
GGDGEDLIE

SEQ ID NO: 34048 - protein, 9 aa, synthetic construct
GGDGEDLIK

SEQ ID NO: 34049 - protein, 9 aa, synthetic construct
GGDGEDLIN

SEQ ID NO: 34050 - protein, 9 aa, synthetic construct
GGDGEDLLF

SEQ ID NO: 34051 - protein, 9 aa, synthetic construct
GGDGEDLLL

SEQ ID NO: 34052 - protein, 9 aa, synthetic construct
GGDGEDLLT

SEQ ID NO: 34053 - protein, 9 aa, synthetic construct
GGDGEDLLV

SEQ ID NO: 34054 - protein, 9 aa, synthetic construct
GGDGEDLMR

SEQ ID NO: 34055 - protein, 9 aa, synthetic construct
GGDGEDLVT

SEQ ID NO: 34056 - protein, 9 aa, synthetic construct
GGDGEDLYI

SEQ ID NO: 34057 - protein, 9 aa, synthetic construct
GGDGEDMLS

SEQ ID NO: 34058 - protein, 9 aa, synthetic construct
GGDGEDQIT

SEQ ID NO: 34059 - protein, 9 aa, synthetic construct
GGDGEDQIY

SEQ ID NO: 34060 - protein, 9 aa, synthetic construct
GGDGEDILF

SEQ ID NO: 34061 - protein, 9 aa, synthetic construct
GGDGEDIIS

SEQ ID NO: 34062 - protein, 9 aa, synthetic construct
GGDGEDQLY

SEQ ID NO: 34063 - protein, 9 aa, synthetic construct
GGDGEDIIA

SEQ ID NO: 34064 - protein, 9 aa, synthetic construct
GGDGEDDLD

SEQ ID NO: 34065 - protein, 9 aa, synthetic construct
GGDGEDDLS

SEQ ID NO: 34066 - protein, 9 aa, synthetic construct
GGDGEDDLY

SEQ ID NO: 34067 - protein, 9 aa, synthetic construct
GGDGEDEIH

SEQ ID NO: 34068 - protein, 9 aa, synthetic construct
GGDGEDELA

SEQ ID NO: 34069 - protein, 9 aa, synthetic construct
GGDGEDELD

SEQ ID NO: 34070 - protein, 9 aa, synthetic construct
GGDGEDELH

SEQ ID NO: 34071 - protein, 9 aa, synthetic construct
GGDGEDEMI

SEQ ID NO: 34072 - protein, 9 aa, synthetic construct
GGDGEDFIG

SEQ ID NO: 34073 - protein, 9 aa, synthetic construct
GGDGEDFIL

SEQ ID NO: 34074 - protein, 9 aa, synthetic construct
GGDGEDFIY

SEQ ID NO: 34075 - protein, 9 aa, synthetic construct
GGDGEDFMN

SEQ ID NO: 34076 - protein, 9 aa, synthetic construct
GGDGEDFVS

SEQ ID NO: 34077 - protein, 9 aa, synthetic construct
GGDGEDGIF

SEQ ID NO: 34078 - protein, 9 aa, synthetic construct
GGDGEDGLF

SEQ ID NO: 34079 - protein, 9 aa, synthetic construct
GGDGEDHLQ

SEQ ID NO: 34080 - protein, 9 aa, synthetic construct
GGDGEDIFV

SEQ ID NO: 34081 - protein, 9 aa, synthetic construct
GGDGEDQLR

SEQ ID NO: 34082 - protein, 9 aa, synthetic construct
GGDGEDRAD

SEQ ID NO: 34083 - protein, 9 aa, synthetic construct
GGDGEDTMR

SEQ ID NO: 34084 - protein, 9 aa, synthetic construct
GGDGEDSLH

SEQ ID NO: 34085 - protein, 9 aa, synthetic construct
GGDGEDSLY

SEQ ID NO: 34086 - protein, 9 aa, synthetic construct
GGDGEDSVL

SEQ ID NO: 34087 - protein, 9 aa, synthetic construct
GGDGEDSVS

SEQ ID NO: 34088 - protein, 9 aa, synthetic construct
GGDGEDTFE

SEQ ID NO: 34089 - protein, 9 aa, synthetic construct
GGDGEDTFH

SEQ ID NO: 34090 - protein, 9 aa, synthetic construct
GGDGEDTIA

SEQ ID NO: 34091 - protein, 9 aa, synthetic construct
GGDGEDTID

SEQ ID NO: 34092 - protein, 9 aa, synthetic construct
GGDGEDTIE

SEQ ID NO: 34093 - protein, 9 aa, synthetic construct
GGDGEDTIF

SEQ ID NO: 34094 - protein, 9 aa, synthetic construct
GGDGEDTIH

SEQ ID NO: 34095 - protein, 9 aa, synthetic construct
GGDGEDTIL

SEQ ID NO: 34096 - protein, 9 aa, synthetic construct
GGDGEDTIR

SEQ ID NO: 34097 - protein, 9 aa, synthetic construct
GGDGEDTIV

SEQ ID NO: 34098 - protein, 9 aa, synthetic construct
GGDGEDTLA

SEQ ID NO: 34099 - protein, 9 aa, synthetic construct
GGDGEDTLG

SEQ ID NO: 34100 - protein, 9 aa, synthetic construct
GGDGEDTLH

SEQ ID NO: 34101 - protein, 9 aa, synthetic construct
GGDGEDTML

SEQ ID NO: 34102 - protein, 9 aa, synthetic construct
GGDGEDSLW

SEQ ID NO: 34103 - protein, 9 aa, synthetic construct
GGDGEDSLD

SEQ ID NO: 34104 - protein, 9 aa, synthetic construct
GGDGEDRIE

SEQ ID NO: 34105 - protein, 9 aa, synthetic construct
GGDGEDSIY

SEQ ID NO: 34106 - protein, 9 aa, synthetic construct
GGDGEDRII

SEQ ID NO: 34107 - protein, 9 aa, synthetic construct
GGDGEDRIL

SEQ ID NO: 34108 - protein, 9 aa, synthetic construct
GGDGEDRIR

SEQ ID NO: 34109 - protein, 9 aa, synthetic construct
GGDGEDRIV

SEQ ID NO: 34110 - protein, 9 aa, synthetic construct
GGDGEDRLD

SEQ ID NO: 34111 - protein, 9 aa, synthetic construct
GGDGEDRLH

SEQ ID NO: 34112 - protein, 9 aa, synthetic construct
GGDGEDRLK

SEQ ID NO: 34113 - protein, 9 aa, synthetic construct
GGDGEDRLM

SEQ ID NO: 34114 - protein, 9 aa, synthetic construct
GGDGEDRLW

SEQ ID NO: 34115 - protein, 9 aa, synthetic construct
GGDGEDRLY

SEQ ID NO: 34116 - protein, 9 aa, synthetic construct
GGDGEDRVE

SEQ ID NO: 34117 - protein, 9 aa, synthetic construct
GGDGEDRVI

SEQ ID NO: 34118 - protein, 9 aa, synthetic construct
GGDGEDSIE

SEQ ID NO: 34119 - protein, 9 aa, synthetic construct
GGDGEDSIF

SEQ ID NO: 34120 - protein, 9 aa, synthetic construct
GGDGEDSIH

SEQ ID NO: 34121 - protein, 9 aa, synthetic construct
GGDGEDSII

SEQ ID NO: 34122 - protein, 9 aa, synthetic construct
GGDGEDSIV

SEQ ID NO: 34123 - protein, 9 aa, synthetic construct
GGEGQDRLQ

SEQ ID NO: 34124 - protein, 9 aa, synthetic construct
GGKGEDTMF

SEQ ID NO: 34125 - protein, 9 aa, synthetic construct
GGEGQDRLY

SEQ ID NO: 34126 - protein, 9 aa, synthetic construct
GGSGADYFH

SEQ ID NO: 34127 - protein, 9 aa, synthetic construct
GGSGADTVH

SEQ ID NO: 34128 - protein, 9 aa, synthetic construct
GGSGADTYA

SEQ ID NO: 34129 - protein, 9 aa, synthetic construct
GGSGADTYF

SEQ ID NO: 34130 - protein, 9 aa, synthetic construct
GGSGADTYI

SEQ ID NO: 34131 - protein, 9 aa, synthetic construct
GGSGADTYK

SEQ ID NO: 34132 - protein, 9 aa, synthetic construct
GGSGADTYL

SEQ ID NO: 34133 - protein, 9 aa, synthetic construct
GGSGADVAV

SEQ ID NO: 34134 - protein, 9 aa, synthetic construct
GGSGADVFD

SEQ ID NO: 34135 - protein, 9 aa, synthetic construct
GGSGADVFF

SEQ ID NO: 34136 - protein, 9 aa, synthetic construct
GGSGADVFM

SEQ ID NO: 34137 - protein, 9 aa, synthetic construct
GGSGADVFN

SEQ ID NO: 34138 - protein, 9 aa, synthetic construct
GGSGADVIN

SEQ ID NO: 34139 - protein, 9 aa, synthetic construct
GGSGADVIR

SEQ ID NO: 34140 - protein, 9 aa, synthetic construct
GGSGADVIV

SEQ ID NO: 34141 - protein, 9 aa, synthetic construct
GGSGADVLA

SEQ ID NO: 34142 - protein, 9 aa, synthetic construct
GGSGADVLE

SEQ ID NO: 34143 - protein, 9 aa, synthetic construct
GGSGADVLH

SEQ ID NO: 34144 - protein, 9 aa, synthetic construct
GGSGADVLM

SEQ ID NO: 34145 - protein, 9 aa, synthetic construct
GGSGADVMD

SEQ ID NO: 34146 - protein, 9 aa, synthetic construct
GGSGADVMH

SEQ ID NO: 34147 - protein, 9 aa, synthetic construct
GGSGADVMK

SEQ ID NO: 34148 - protein, 9 aa, synthetic construct
GGSGADVMY

SEQ ID NO: 34149 - protein, 9 aa, synthetic construct
GGSGADVVR

SEQ ID NO: 34150 - protein, 9 aa, synthetic construct
GGSGADVYE

SEQ ID NO: 34151 - protein, 9 aa, synthetic construct
GGSGADWLF

SEQ ID NO: 34152 - protein, 9 aa, synthetic construct
GGSGADWLI

SEQ ID NO: 34153 - protein, 9 aa, synthetic construct
GGSGADWLN

SEQ ID NO: 34154 - protein, 9 aa, synthetic construct
GGSGADWLR

SEQ ID NO: 34155 - protein, 9 aa, synthetic construct
GGSGADWVD

SEQ ID NO: 34156 - protein, 9 aa, synthetic construct
GGSGADTMW

SEQ ID NO: 34157 - protein, 9 aa, synthetic construct
GGSGADTMN

SEQ ID NO: 34158 - protein, 9 aa, synthetic construct
GGSGADTMF

SEQ ID NO: 34159 - protein, 9 aa, synthetic construct
GGSGADSVA

SEQ ID NO: 34160 - protein, 9 aa, synthetic construct
GGSGADSFE

SEQ ID NO: 34161 - protein, 9 aa, synthetic construct
GGSGADSFH

SEQ ID NO: 34162 - protein, 9 aa, synthetic construct
GGSGADSFR

SEQ ID NO: 34163 - protein, 9 aa, synthetic construct
GGSGADSII

SEQ ID NO: 34164 - protein, 9 aa, synthetic construct
GGSGADSIV

SEQ ID NO: 34165 - protein, 9 aa, synthetic construct
GGSGADSIY

SEQ ID NO: 34166 - protein, 9 aa, synthetic construct
GGSGADSLF

SEQ ID NO: 34167 - protein, 9 aa, synthetic construct
GGSGADSLM

SEQ ID NO: 34168 - protein, 9 aa, synthetic construct
GGSGADSLR

SEQ ID NO: 34169 - protein, 9 aa, synthetic construct
GGSGADSLW

SEQ ID NO: 34170 - protein, 9 aa, synthetic construct
GGSGADSMD

SEQ ID NO: 34171 - protein, 9 aa, synthetic construct
GGSGADSML

SEQ ID NO: 34172 - protein, 9 aa, synthetic construct
GGSGADSMN

SEQ ID NO: 34173 - protein, 9 aa, synthetic construct
GGSGADSVH

SEQ ID NO: 34174 - protein, 9 aa, synthetic construct
GGSGADTIM

SEQ ID NO: 34175 - protein, 9 aa, synthetic construct
GGSGADSVI

SEQ ID NO: 34176 - protein, 9 aa, synthetic construct
GGSGADSVS

SEQ ID NO: 34177 - protein, 9 aa, synthetic construct
GGSGADSYY

SEQ ID NO: 34178 - protein, 9 aa, synthetic construct
GGSGADTAA

SEQ ID NO: 34179 - protein, 9 aa, synthetic construct
GGSGADTAE

SEQ ID NO: 34180 - protein, 9 aa, synthetic construct
GGSGADTAF

SEQ ID NO: 34181 - protein, 9 aa, synthetic construct
GGSGADTAS

SEQ ID NO: 34182 - protein, 9 aa, synthetic construct
GGSGADTAY

SEQ ID NO: 34183 - protein, 9 aa, synthetic construct
GGSGADTFN

SEQ ID NO: 34184 - protein, 9 aa, synthetic construct
GGSGADTFS

SEQ ID NO: 34185 - protein, 9 aa, synthetic construct
GGSGADTFW

SEQ ID NO: 34186 - protein, 9 aa, synthetic construct
GGSGADTIH

SEQ ID NO: 34187 - protein, 9 aa, synthetic construct
GGSGADTIK

SEQ ID NO: 34188 - protein, 9 aa, synthetic construct
GGSGADYAE

SEQ ID NO: 34189 - protein, 9 aa, synthetic construct
GGSGADYFV

SEQ ID NO: 34190 - protein, 9 aa, synthetic construct
GGSGDDEVK

SEQ ID NO: 34191 - protein, 9 aa, synthetic construct
GGSGADYIV

SEQ ID NO: 34192 - protein, 9 aa, synthetic construct
GGSGDDAVT

SEQ ID NO: 34193 - protein, 9 aa, synthetic construct
GGSGDDAVY

SEQ ID NO: 34194 - protein, 9 aa, synthetic construct
GGSGDDAYF

SEQ ID NO: 34195 - protein, 9 aa, synthetic construct
GGSGDDAYH

SEQ ID NO: 34196 - protein, 9 aa, synthetic construct
GGSGDDAYM

SEQ ID NO: 34197 - protein, 9 aa, synthetic construct
GGSGDDCIL

SEQ ID NO: 34198 - protein, 9 aa, synthetic construct
GGSGDDCLF

SEQ ID NO: 34199 - protein, 9 aa, synthetic construct
GGSGDDDAF

SEQ ID NO: 34200 - protein, 9 aa, synthetic construct
GGSGDDDID

SEQ ID NO: 34201 - protein, 9 aa, synthetic construct
GGSGDDDIH

SEQ ID NO: 34202 - protein, 9 aa, synthetic construct
GGSGDDDIK

SEQ ID NO: 34203 - protein, 9 aa, synthetic construct
GGSGDDDIS

SEQ ID NO: 34204 - protein, 9 aa, synthetic construct
GGSGDDDMD

SEQ ID NO: 34205 - protein, 9 aa, synthetic construct
GGSGDDDMI

SEQ ID NO: 34206 - protein, 9 aa, synthetic construct
GGSGDDDVL

SEQ ID NO: 34207 - protein, 9 aa, synthetic construct
GGSGDDDVS

SEQ ID NO: 34208 - protein, 9 aa, synthetic construct
GGSGDDEAQ

SEQ ID NO: 34209 - protein, 9 aa, synthetic construct
GGSGDDEIG

SEQ ID NO: 34210 - protein, 9 aa, synthetic construct
GGSGDDEIH

SEQ ID NO: 34211 - protein, 9 aa, synthetic construct
GGSGDDEIL

SEQ ID NO: 34212 - protein, 9 aa, synthetic construct
GGSGDDEIM

SEQ ID NO: 34213 - protein, 9 aa, synthetic construct
GGSGDDEIR

SEQ ID NO: 34214 - protein, 9 aa, synthetic construct
GGSGDDELE

SEQ ID NO: 34215 - protein, 9 aa, synthetic construct
GGSGDDELQ

SEQ ID NO: 34216 - protein, 9 aa, synthetic construct
GGSGDDELW

SEQ ID NO: 34217 - protein, 9 aa, synthetic construct
GGSGDDEMH

SEQ ID NO: 34218 - protein, 9 aa, synthetic construct
GGSGDDEMT

SEQ ID NO: 34219 - protein, 9 aa, synthetic construct
GGSGDDEMY

SEQ ID NO: 34220 - protein, 9 aa, synthetic construct
GGSGDDEVD

SEQ ID NO: 34221 - protein, 9 aa, synthetic construct
GGSGDDAVN

SEQ ID NO: 34222 - protein, 9 aa, synthetic construct
GGSGDDAVI

SEQ ID NO: 34223 - protein, 9 aa, synthetic construct
GGSGDDAVA

SEQ ID NO: 34224 - protein, 9 aa, synthetic construct
GGSGADYVD

SEQ ID NO: 34225 - protein, 9 aa, synthetic construct
GGSGADYLA

SEQ ID NO: 34226 - protein, 9 aa, synthetic construct
GGSGADYLE

SEQ ID NO: 34227 - protein, 9 aa, synthetic construct
GGSGADYLH

SEQ ID NO: 34228 - protein, 9 aa, synthetic construct
GGSGADYLL

SEQ ID NO: 34229 - protein, 9 aa, synthetic construct
GGSGADYLQ

SEQ ID NO: 34230 - protein, 9 aa, synthetic construct
GGSGADYLT

SEQ ID NO: 34231 - protein, 9 aa, synthetic construct
GGSGADYLY

SEQ ID NO: 34232 - protein, 9 aa, synthetic construct
GGSGADYMD

SEQ ID NO: 34233 - protein, 9 aa, synthetic construct
GGSGADYME

SEQ ID NO: 34234 - protein, 9 aa, synthetic construct
GGSGADYMK

SEQ ID NO: 34235 - protein, 9 aa, synthetic construct
GGSGADYMR

SEQ ID NO: 34236 - protein, 9 aa, synthetic construct
GGSGADYMT

SEQ ID NO: 34237 - protein, 9 aa, synthetic construct
GGSGADYMW

SEQ ID NO: 34238 - protein, 9 aa, synthetic construct
GGSGCDKID

SEQ ID NO: 34239 - protein, 9 aa, synthetic construct
GGSGDDAMW

SEQ ID NO: 34240 - protein, 9 aa, synthetic construct
GGSGCDSLD

SEQ ID NO: 34241 - protein, 9 aa, synthetic construct
GGSGCDTLN

SEQ ID NO: 34242 - protein, 9 aa, synthetic construct
GGSGCDVMA

SEQ ID NO: 34243 - protein, 9 aa, synthetic construct
GGSGDDAFV

SEQ ID NO: 34244 - protein, 9 aa, synthetic construct
GGSGDDAIT

SEQ ID NO: 34245 - protein, 9 aa, synthetic construct
GGSGDDAIV

SEQ ID NO: 34246 - protein, 9 aa, synthetic construct
GGSGDDAIW

SEQ ID NO: 34247 - protein, 9 aa, synthetic construct
GGSGDDALK

SEQ ID NO: 34248 - protein, 9 aa, synthetic construct
GGSGDDALL

SEQ ID NO: 34249 - protein, 9 aa, synthetic construct
GGSGDDALM

SEQ ID NO: 34250 - protein, 9 aa, synthetic construct
GGSGDDAMD

SEQ ID NO: 34251 - protein, 9 aa, synthetic construct
GGSGDDAME

SEQ ID NO: 34252 - protein, 9 aa, synthetic construct
GGSGDDAML

SEQ ID NO: 34253 - protein, 9 aa, synthetic construct
GGSGADSFD

SEQ ID NO: 34254 - protein, 9 aa, synthetic construct
GGSGADSFC

SEQ ID NO: 34255 - protein, 9 aa, synthetic construct
GGSGADRVN

SEQ ID NO: 34256 - protein, 9 aa, synthetic construct
GGSGADRVF

SEQ ID NO: 34257 - protein, 9 aa, synthetic construct
GGSGADIMH

SEQ ID NO: 34258 - protein, 9 aa, synthetic construct
GGSGADIMS

SEQ ID NO: 34259 - protein, 9 aa, synthetic construct
GGSGADIMY

SEQ ID NO: 34260 - protein, 9 aa, synthetic construct
GGSGADIVL

SEQ ID NO: 34261 - protein, 9 aa, synthetic construct
GGSGADIVQ

SEQ ID NO: 34262 - protein, 9 aa, synthetic construct
GGSGADIVS

SEQ ID NO: 34263 - protein, 9 aa, synthetic construct
GGSGADIYL

SEQ ID NO: 34264 - protein, 9 aa, synthetic construct
GGSGADKFA

SEQ ID NO: 34265 - protein, 9 aa, synthetic construct
GGSGADKFF

SEQ ID NO: 34266 - protein, 9 aa, synthetic construct
GGSGADKFK

SEQ ID NO: 34267 - protein, 9 aa, synthetic construct
GGSGADKIA

SEQ ID NO: 34268 - protein, 9 aa, synthetic construct
GGSGADKIS

SEQ ID NO: 34269 - protein, 9 aa, synthetic construct
GGSGADKIT

SEQ ID NO: 34270 - protein, 9 aa, synthetic construct
GGSGADKLD

SEQ ID NO: 34271 - protein, 9 aa, synthetic construct
GGSGADKLF

SEQ ID NO: 34272 - protein, 9 aa, synthetic construct
GGSGADKLW

SEQ ID NO: 34273 - protein, 9 aa, synthetic construct
GGSGADKMD

SEQ ID NO: 34274 - protein, 9 aa, synthetic construct
GGSGADKVA

SEQ ID NO: 34275 - protein, 9 aa, synthetic construct
GGSGADKVY

SEQ ID NO: 34276 - protein, 9 aa, synthetic construct
GGSGADKYI

SEQ ID NO: 34277 - protein, 9 aa, synthetic construct
GGSGADLAC

SEQ ID NO: 34278 - protein, 9 aa, synthetic construct
GGSGADLAF

SEQ ID NO: 34279 - protein, 9 aa, synthetic construct
GGSGADLAH

SEQ ID NO: 34280 - protein, 9 aa, synthetic construct
GGSGADLAY

SEQ ID NO: 34281 - protein, 9 aa, synthetic construct
GGSGADLFC

SEQ ID NO: 34282 - protein, 9 aa, synthetic construct
GGSGADLFD

SEQ ID NO: 34283 - protein, 9 aa, synthetic construct
GGSGADLFF

SEQ ID NO: 34284 - protein, 9 aa, synthetic construct
GGSGADLFL

SEQ ID NO: 34285 - protein, 9 aa, synthetic construct
GGSGADLFT

SEQ ID NO: 34286 - protein, 9 aa, synthetic construct
GGSGADIMF

SEQ ID NO: 34287 - protein, 9 aa, synthetic construct
GGSGADIMD

SEQ ID NO: 34288 - protein, 9 aa, synthetic construct
GGSGADILY

SEQ ID NO: 34289 - protein, 9 aa, synthetic construct
GGSGADHLA

SEQ ID NO: 34290 - protein, 9 aa, synthetic construct
GGSGADFMG

SEQ ID NO: 34291 - protein, 9 aa, synthetic construct
GGSGADFMQ

SEQ ID NO: 34292 - protein, 9 aa, synthetic construct
GGSGADFMR

SEQ ID NO: 34293 - protein, 9 aa, synthetic construct
GGSGADFVN

SEQ ID NO: 34294 - protein, 9 aa, synthetic construct
GGSGADGFI

SEQ ID NO: 34295 - protein, 9 aa, synthetic construct
GGSGADGFY

SEQ ID NO: 34296 - protein, 9 aa, synthetic construct
GGSGADGLD

SEQ ID NO: 34297 - protein, 9 aa, synthetic construct
GGSGADGLN

SEQ ID NO: 34298 - protein, 9 aa, synthetic construct
GGSGADGLY

SEQ ID NO: 34299 - protein, 9 aa, synthetic construct
GGSGADGVY

SEQ ID NO: 34300 - protein, 9 aa, synthetic construct
GGSGADHFI

SEQ ID NO: 34301 - protein, 9 aa, synthetic construct
GGSGADHFL

SEQ ID NO: 34302 - protein, 9 aa, synthetic construct
GGSGADHFN

SEQ ID NO: 34303 - protein, 9 aa, synthetic construct
GGSGADHLE

SEQ ID NO: 34304 - protein, 9 aa, synthetic construct
GGSGADILQ

SEQ ID NO: 34305 - protein, 9 aa, synthetic construct
GGSGADHLF

SEQ ID NO: 34306 - protein, 9 aa, synthetic construct
GGSGADHLQ

SEQ ID NO: 34307 - protein, 9 aa, synthetic construct
GGSGADHLY

SEQ ID NO: 34308 - protein, 9 aa, synthetic construct
GGSGADIAV

SEQ ID NO: 34309 - protein, 9 aa, synthetic construct
GGSGADIAY

SEQ ID NO: 34310 - protein, 9 aa, synthetic construct
GGSGADIFS

SEQ ID NO: 34311 - protein, 9 aa, synthetic construct
GGSGADIIH

SEQ ID NO: 34312 - protein, 9 aa, synthetic construct
GGSGADIII

SEQ ID NO: 34313 - protein, 9 aa, synthetic construct
GGSGADIIL

SEQ ID NO: 34314 - protein, 9 aa, synthetic construct
GGSGADIIV

SEQ ID NO: 34315 - protein, 9 aa, synthetic construct
GGSGADILA

SEQ ID NO: 34316 - protein, 9 aa, synthetic construct
GGSGADILG

SEQ ID NO: 34317 - protein, 9 aa, synthetic construct
GGSGADILM

SEQ ID NO: 34318 - protein, 9 aa, synthetic construct
GGSGADLID

SEQ ID NO: 34319 - protein, 9 aa, synthetic construct
GGSGADLIE

SEQ ID NO: 34320 - protein, 9 aa, synthetic construct
GGSGADLIG

SEQ ID NO: 34321 - protein, 9 aa, synthetic construct
GGSGADRFW

SEQ ID NO: 34322 - protein, 9 aa, synthetic construct
GGSGADQID

SEQ ID NO: 34323 - protein, 9 aa, synthetic construct
GGSGADQLH

SEQ ID NO: 34324 - protein, 9 aa, synthetic construct
GGSGADQLL

SEQ ID NO: 34325 - protein, 9 aa, synthetic construct
GGSGADQLR

SEQ ID NO: 34326 - protein, 9 aa, synthetic construct
GGSGADQMF

SEQ ID NO: 34327 - protein, 9 aa, synthetic construct
GGSGADQMH

SEQ ID NO: 34328 - protein, 9 aa, synthetic construct
GGSGADQMR

SEQ ID NO: 34329 - protein, 9 aa, synthetic construct
GGSGADQMS

SEQ ID NO: 34330 - protein, 9 aa, synthetic construct
GGSGADQMW

SEQ ID NO: 34331 - protein, 9 aa, synthetic construct
GGSGADQVI

SEQ ID NO: 34332 - protein, 9 aa, synthetic construct
GGSGADRFA

SEQ ID NO: 34333 - protein, 9 aa, synthetic construct
GGSGADRFK

SEQ ID NO: 34334 - protein, 9 aa, synthetic construct
GGSGADRFT

SEQ ID NO: 34335 - protein, 9 aa, synthetic construct
GGSGADRIF

SEQ ID NO: 34336 - protein, 9 aa, synthetic construct
GGSGADQFK

SEQ ID NO: 34337 - protein, 9 aa, synthetic construct
GGSGADRIH

SEQ ID NO: 34338 - protein, 9 aa, synthetic construct
GGSGADRIL

SEQ ID NO: 34339 - protein, 9 aa, synthetic construct
GGSGADRIS

SEQ ID NO: 34340 - protein, 9 aa, synthetic construct
GGSGADRIY

SEQ ID NO: 34341 - protein, 9 aa, synthetic construct
GGSGADRLG

SEQ ID NO: 34342 - protein, 9 aa, synthetic construct
GGSGADRLQ

SEQ ID NO: 34343 - protein, 9 aa, synthetic construct
GGSGADRLR

SEQ ID NO: 34344 - protein, 9 aa, synthetic construct
GGSGADRMF

SEQ ID NO: 34345 - protein, 9 aa, synthetic construct
GGSGADRMH

SEQ ID NO: 34346 - protein, 9 aa, synthetic construct
GGSGADRMS

SEQ ID NO: 34347 - protein, 9 aa, synthetic construct
GGSGADRMV

SEQ ID NO: 34348 - protein, 9 aa, synthetic construct
GGSGADRMW

SEQ ID NO: 34349 - protein, 9 aa, synthetic construct
GGSGADRVD

SEQ ID NO: 34350 - protein, 9 aa, synthetic construct
GGSGADQIA

SEQ ID NO: 34351 - protein, 9 aa, synthetic construct
GGSGADNYV

SEQ ID NO: 34352 - protein, 9 aa, synthetic construct
GGSGADLIL

SEQ ID NO: 34353 - protein, 9 aa, synthetic construct
GGSGADMIE

SEQ ID NO: 34354 - protein, 9 aa, synthetic construct
GGSGADLIT

SEQ ID NO: 34355 - protein, 9 aa, synthetic construct
GGSGADLMQ

SEQ ID NO: 34356 - protein, 9 aa, synthetic construct
GGSGADLMR

SEQ ID NO: 34357 - protein, 9 aa, synthetic construct
GGSGADLVQ

SEQ ID NO: 34358 - protein, 9 aa, synthetic construct
GGSGADLVT

SEQ ID NO: 34359 - protein, 9 aa, synthetic construct
GGSGADLVY

SEQ ID NO: 34360 - protein, 9 aa, synthetic construct
GGSGADMAN

SEQ ID NO: 34361 - protein, 9 aa, synthetic construct
GGSGADMFD

SEQ ID NO: 34362 - protein, 9 aa, synthetic construct
GGSGADMFF

SEQ ID NO: 34363 - protein, 9 aa, synthetic construct
GGSGADMFL

SEQ ID NO: 34364 - protein, 9 aa, synthetic construct
GGSGADMFQ

SEQ ID NO: 34365 - protein, 9 aa, synthetic construct
GGSGADMFV

SEQ ID NO: 34366 - protein, 9 aa, synthetic construct
GGSGADMID

SEQ ID NO: 34367 - protein, 9 aa, synthetic construct
GGSGADMIR

SEQ ID NO: 34368 - protein, 9 aa, synthetic construct
GGSGADNVD

SEQ ID NO: 34369 - protein, 9 aa, synthetic construct
GGSGADMLE

SEQ ID NO: 34370 - protein, 9 aa, synthetic construct
GGSGADMLH

SEQ ID NO: 34371 - protein, 9 aa, synthetic construct
GGSGADMLS

SEQ ID NO: 34372 - protein, 9 aa, synthetic construct
GGSGADMMI

SEQ ID NO: 34373 - protein, 9 aa, synthetic construct
GGSGADNFM

SEQ ID NO: 34374 - protein, 9 aa, synthetic construct
GGSGADNID

SEQ ID NO: 34375 - protein, 9 aa, synthetic construct
GGSGADNIF

SEQ ID NO: 34376 - protein, 9 aa, synthetic construct
GGSGADNIK

SEQ ID NO: 34377 - protein, 9 aa, synthetic construct
GGSGADNLG

SEQ ID NO: 34378 - protein, 9 aa, synthetic construct
GGSGADNLL

SEQ ID NO: 34379 - protein, 9 aa, synthetic construct
GGSGADNLW

SEQ ID NO: 34380 - protein, 9 aa, synthetic construct
GGSGADNMF

SEQ ID NO: 34381 - protein, 9 aa, synthetic construct
GGSGADNMT

SEQ ID NO: 34382 - protein, 9 aa, synthetic construct
GGSGDDEVH

SEQ ID NO: 34383 - protein, 9 aa, synthetic construct
GGSGDDFFD

SEQ ID NO: 34384 - protein, 9 aa, synthetic construct
GGSGADFLR

SEQ ID NO: 34385 - protein, 9 aa, synthetic construct
GGSGDDVIG

SEQ ID NO: 34386 - protein, 9 aa, synthetic construct
GGSGDDTAD

SEQ ID NO: 34387 - protein, 9 aa, synthetic construct
GGSGDDTAG

SEQ ID NO: 34388 - protein, 9 aa, synthetic construct
GGSGDDTAK

SEQ ID NO: 34389 - protein, 9 aa, synthetic construct
GGSGDDTAS

SEQ ID NO: 34390 - protein, 9 aa, synthetic construct
GGSGDDTAY

SEQ ID NO: 34391 - protein, 9 aa, synthetic construct
GGSGDDTFD

SEQ ID NO: 34392 - protein, 9 aa, synthetic construct
GGSGDDTFF

SEQ ID NO: 34393 - protein, 9 aa, synthetic construct
GGSGDDTFN

SEQ ID NO: 34394 - protein, 9 aa, synthetic construct
GGSGDDTFW

SEQ ID NO: 34395 - protein, 9 aa, synthetic construct
GGSGDDTMD

SEQ ID NO: 34396 - protein, 9 aa, synthetic construct
GGSGDDTMF

SEQ ID NO: 34397 - protein, 9 aa, synthetic construct
GGSGDDTMH

SEQ ID NO: 34398 - protein, 9 aa, synthetic construct
GGSGDDTMI

SEQ ID NO: 34399 - protein, 9 aa, synthetic construct
GGSGDDTMN

SEQ ID NO: 34400 - protein, 9 aa, synthetic construct
GGSGDDTMQ

SEQ ID NO: 34401 - protein, 9 aa, synthetic construct
GGSGDDTMY

SEQ ID NO: 34402 - protein, 9 aa, synthetic construct
GGSGDDTVH

SEQ ID NO: 34403 - protein, 9 aa, synthetic construct
GGSGDDTVQ

SEQ ID NO: 34404 - protein, 9 aa, synthetic construct
GGSGDDTVV

SEQ ID NO: 34405 - protein, 9 aa, synthetic construct
GGSGDDTYA

SEQ ID NO: 34406 - protein, 9 aa, synthetic construct
GGSGDDVAD

SEQ ID NO: 34407 - protein, 9 aa, synthetic construct
GGSGDDVAE

SEQ ID NO: 34408 - protein, 9 aa, synthetic construct
GGSGDDVAL

SEQ ID NO: 34409 - protein, 9 aa, synthetic construct
GGSGDDVAM

SEQ ID NO: 34410 - protein, 9 aa, synthetic construct
GGSGDDVAS

SEQ ID NO: 34411 - protein, 9 aa, synthetic construct
GGSGDDVAY

SEQ ID NO: 34412 - protein, 9 aa, synthetic construct
GGSGDDVFA

SEQ ID NO: 34413 - protein, 9 aa, synthetic construct
GGSGDDVFH

SEQ ID NO: 34414 - protein, 9 aa, synthetic construct
GGSGDDVFK

SEQ ID NO: 34415 - protein, 9 aa, synthetic construct
GGSGDDSYW

SEQ ID NO: 34416 - protein, 9 aa, synthetic construct
GGSGDDSYT

SEQ ID NO: 34417 - protein, 9 aa, synthetic construct
GGSGDDSYK

SEQ ID NO: 34418 - protein, 9 aa, synthetic construct
GGSGDDSAD

SEQ ID NO: 34419 - protein, 9 aa, synthetic construct
GGSGDDRMA

SEQ ID NO: 34420 - protein, 9 aa, synthetic construct
GGSGDDRMH

SEQ ID NO: 34421 - protein, 9 aa, synthetic construct
GGSGDDRMT

SEQ ID NO: 34422 - protein, 9 aa, synthetic construct
GGSGDDRMV

SEQ ID NO: 34423 - protein, 9 aa, synthetic construct
GGSGDDRMW

SEQ ID NO: 34424 - protein, 9 aa, synthetic construct
GGSGDDRVD

SEQ ID NO: 34425 - protein, 9 aa, synthetic construct
GGSGDDRVH

SEQ ID NO: 34426 - protein, 9 aa, synthetic construct
GGSGDDRVL

SEQ ID NO: 34427 - protein, 9 aa, synthetic construct
GGSGDDRVR

SEQ ID NO: 34428 - protein, 9 aa, synthetic construct
GGSGDDRYA

SEQ ID NO: 34429 - protein, 9 aa, synthetic construct
GGSGDDRYF

SEQ ID NO: 34430 - protein, 9 aa, synthetic construct
GGSGDDRYL

SEQ ID NO: 34431 - protein, 9 aa, synthetic construct
GGSGDDRYV

SEQ ID NO: 34432 - protein, 9 aa, synthetic construct
GGSGDDSAQ

SEQ ID NO: 34433 - protein, 9 aa, synthetic construct
GGSGDDSVG

SEQ ID NO: 34434 - protein, 9 aa, synthetic construct
GGSGDDSFG

SEQ ID NO: 34435 - protein, 9 aa, synthetic construct
GGSGDDSFK

SEQ ID NO: 34436 - protein, 9 aa, synthetic construct
GGSGDDSFS

SEQ ID NO: 34437 - protein, 9 aa, synthetic construct
GGSGDDSFV

SEQ ID NO: 34438 - protein, 9 aa, synthetic construct
GGSGDDSFY

SEQ ID NO: 34439 - protein, 9 aa, synthetic construct
GGSGDDSIF

SEQ ID NO: 34440 - protein, 9 aa, synthetic construct
GGSGDDSIK

SEQ ID NO: 34441 - protein, 9 aa, synthetic construct
GGSGDDSIV

SEQ ID NO: 34442 - protein, 9 aa, synthetic construct
GGSGDDSLK

SEQ ID NO: 34443 - protein, 9 aa, synthetic construct
GGSGDDSMD

SEQ ID NO: 34444 - protein, 9 aa, synthetic construct
GGSGDDSML

SEQ ID NO: 34445 - protein, 9 aa, synthetic construct
GGSGDDSMT

SEQ ID NO: 34446 - protein, 9 aa, synthetic construct
GGSGDDSVD

SEQ ID NO: 34447 - protein, 9 aa, synthetic construct
GGSGDDVIF

SEQ ID NO: 34448 - protein, 9 aa, synthetic construct
GGSGDDVIM

SEQ ID NO: 34449 - protein, 9 aa, synthetic construct
GGSGDDFIA

SEQ ID NO: 34450 - protein, 9 aa, synthetic construct
GGSGDDVIR

SEQ ID NO: 34451 - protein, 9 aa, synthetic construct
GGSGDDYIV

SEQ ID NO: 34452 - protein, 9 aa, synthetic construct
GGSGDDYIY

SEQ ID NO: 34453 - protein, 9 aa, synthetic construct
GGSGDDYLM

SEQ ID NO: 34454 - protein, 9 aa, synthetic construct
GGSGDDYLT

SEQ ID NO: 34455 - protein, 9 aa, synthetic construct
GGSGDDYMD

SEQ ID NO: 34456 - protein, 9 aa, synthetic construct
GGSGDDYMY

SEQ ID NO: 34457 - protein, 9 aa, synthetic construct
GGSGDDYVD

SEQ ID NO: 34458 - protein, 9 aa, synthetic construct
GGSGDDYVY

SEQ ID NO: 34459 - protein, 9 aa, synthetic construct
GGSGEDALA

SEQ ID NO: 34460 - protein, 9 aa, synthetic construct
GGSGEDALW

SEQ ID NO: 34461 - protein, 9 aa, synthetic construct
GGSGEDALY

SEQ ID NO: 34462 - protein, 9 aa, synthetic construct
GGSGEDAMF

SEQ ID NO: 34463 - protein, 9 aa, synthetic construct
GGSGEDCAD

SEQ ID NO: 34464 - protein, 9 aa, synthetic construct
GGSGEDDIN

SEQ ID NO: 34465 - protein, 9 aa, synthetic construct
GGSGEDDIV

SEQ ID NO: 34466 - protein, 9 aa, synthetic construct
GGSGEDDLF

SEQ ID NO: 34467 - protein, 9 aa, synthetic construct
GGSGEDDLH

SEQ ID NO: 34468 - protein, 9 aa, synthetic construct
GGSGEDEIL

SEQ ID NO: 34469 - protein, 9 aa, synthetic construct
GGSGEDELS

SEQ ID NO: 34470 - protein, 9 aa, synthetic construct
GGSGEDEMH

SEQ ID NO: 34471 - protein, 9 aa, synthetic construct
GGSGEDFFV

SEQ ID NO: 34472 - protein, 9 aa, synthetic construct
GGSGEDFIQ

SEQ ID NO: 34473 - protein, 9 aa, synthetic construct
GGSGEDFIR

SEQ ID NO: 34474 - protein, 9 aa, synthetic construct
GGSGEDFLN

SEQ ID NO: 34475 - protein, 9 aa, synthetic construct
GGSGEDFLS

SEQ ID NO: 34476 - protein, 9 aa, synthetic construct
GGSGEDFLY

SEQ ID NO: 34477 - protein, 9 aa, synthetic construct
GGSGEDGIV

SEQ ID NO: 34478 - protein, 9 aa, synthetic construct
GGSGEDHFW

SEQ ID NO: 34479 - protein, 9 aa, synthetic construct
GGSGEDHLA

SEQ ID NO: 34480 - protein, 9 aa, synthetic construct
GGSGDDYIR

SEQ ID NO: 34481 - protein, 9 aa, synthetic construct
GGSGDDYIN

SEQ ID NO: 34482 - protein, 9 aa, synthetic construct
GGSGDDYIE

SEQ ID NO: 34483 - protein, 9 aa, synthetic construct
GGSGDDWIA

SEQ ID NO: 34484 - protein, 9 aa, synthetic construct
GGSGDDVME

SEQ ID NO: 34485 - protein, 9 aa, synthetic construct
GGSGDDVMF

SEQ ID NO: 34486 - protein, 9 aa, synthetic construct
GGSGDDVMR

SEQ ID NO: 34487 - protein, 9 aa, synthetic construct
GGSGDDVMV

SEQ ID NO: 34488 - protein, 9 aa, synthetic construct
GGSGDDVVE

SEQ ID NO: 34489 - protein, 9 aa, synthetic construct
GGSGDDVVI

SEQ ID NO: 34490 - protein, 9 aa, synthetic construct
GGSGDDVVL

SEQ ID NO: 34491 - protein, 9 aa, synthetic construct
GGSGDDVVM

SEQ ID NO: 34492 - protein, 9 aa, synthetic construct
GGSGDDVVN

SEQ ID NO: 34493 - protein, 9 aa, synthetic construct
GGSGDDVVT

SEQ ID NO: 34494 - protein, 9 aa, synthetic construct
GGSGDDVVW

SEQ ID NO: 34495 - protein, 9 aa, synthetic construct
GGSGDDVYF

SEQ ID NO: 34496 - protein, 9 aa, synthetic construct
GGSGDDVYR

SEQ ID NO: 34497 - protein, 9 aa, synthetic construct
GGSGDDWIH

SEQ ID NO: 34498 - protein, 9 aa, synthetic construct
GGSGDDYIA

SEQ ID NO: 34499 - protein, 9 aa, synthetic construct
GGSGDDWIL

SEQ ID NO: 34500 - protein, 9 aa, synthetic construct
GGSGDDWLN

SEQ ID NO: 34501 - protein, 9 aa, synthetic construct
GGSGDDWLQ

SEQ ID NO: 34502 - protein, 9 aa, synthetic construct
GGSGDDWLY

SEQ ID NO: 34503 - protein, 9 aa, synthetic construct
GGSGDDWME

SEQ ID NO: 34504 - protein, 9 aa, synthetic construct
GGSGDDWMR

SEQ ID NO: 34505 - protein, 9 aa, synthetic construct
GGSGDDWMS

SEQ ID NO: 34506 - protein, 9 aa, synthetic construct
GGSGDDWMV

SEQ ID NO: 34507 - protein, 9 aa, synthetic construct
GGSGDDWVD

SEQ ID NO: 34508 - protein, 9 aa, synthetic construct
GGSGDDWVI

SEQ ID NO: 34509 - protein, 9 aa, synthetic construct
GGSGDDYAD

SEQ ID NO: 34510 - protein, 9 aa, synthetic construct
GGSGDDYFD

SEQ ID NO: 34511 - protein, 9 aa, synthetic construct
GGSGDDYFQ

SEQ ID NO: 34512 - protein, 9 aa, synthetic construct
GGSGDDRLQ

SEQ ID NO: 34513 - protein, 9 aa, synthetic construct
GGSGDDRLK

SEQ ID NO: 34514 - protein, 9 aa, synthetic construct
GGSGDDRIH

SEQ ID NO: 34515 - protein, 9 aa, synthetic construct
GGSGDDRFY

SEQ ID NO: 34516 - protein, 9 aa, synthetic construct
GGSGDDIFG

SEQ ID NO: 34517 - protein, 9 aa, synthetic construct
GGSGDDIFS

SEQ ID NO: 34518 - protein, 9 aa, synthetic construct
GGSGDDIFY

SEQ ID NO: 34519 - protein, 9 aa, synthetic construct
GGSGDDIIM

SEQ ID NO: 34520 - protein, 9 aa, synthetic construct
GGSGDDIMA

SEQ ID NO: 34521 - protein, 9 aa, synthetic construct
GGSGDDIMK

SEQ ID NO: 34522 - protein, 9 aa, synthetic construct
GGSGDDIMR

SEQ ID NO: 34523 - protein, 9 aa, synthetic construct
GGSGDDIMY

SEQ ID NO: 34524 - protein, 9 aa, synthetic construct
GGSGDDIVE

SEQ ID NO: 34525 - protein, 9 aa, synthetic construct
GGSGDDIVI

SEQ ID NO: 34526 - protein, 9 aa, synthetic construct
GGSGDDIVS

SEQ ID NO: 34527 - protein, 9 aa, synthetic construct
GGSGDDIVV

SEQ ID NO: 34528 - protein, 9 aa, synthetic construct
GGSGDDIYF

SEQ ID NO: 34529 - protein, 9 aa, synthetic construct
GGSGDDIYQ

SEQ ID NO: 34530 - protein, 9 aa, synthetic construct
GGSGDDKFD

SEQ ID NO: 34531 - protein, 9 aa, synthetic construct
GGSGDDKFF

SEQ ID NO: 34532 - protein, 9 aa, synthetic construct
GGSGDDKFI

SEQ ID NO: 34533 - protein, 9 aa, synthetic construct
GGSGDDKFW

SEQ ID NO: 34534 - protein, 9 aa, synthetic construct
GGSGDDKIA

SEQ ID NO: 34535 - protein, 9 aa, synthetic construct
GGSGDDKIF

SEQ ID NO: 34536 - protein, 9 aa, synthetic construct
GGSGDDKIG

SEQ ID NO: 34537 - protein, 9 aa, synthetic construct
GGSGDDKIL

SEQ ID NO: 34538 - protein, 9 aa, synthetic construct
GGSGDDKIV

SEQ ID NO: 34539 - protein, 9 aa, synthetic construct
GGSGDDKLI

SEQ ID NO: 34540 - protein, 9 aa, synthetic construct
GGSGDDKLK

SEQ ID NO: 34541 - protein, 9 aa, synthetic construct
GGSGDDKLT

SEQ ID NO: 34542 - protein, 9 aa, synthetic construct
GGSGDDKMV

SEQ ID NO: 34543 - protein, 9 aa, synthetic construct
GGSGDDKMY

SEQ ID NO: 34544 - protein, 9 aa, synthetic construct
GGSGDDKYV

SEQ ID NO: 34545 - protein, 9 aa, synthetic construct
GGSGDDIFE

SEQ ID NO: 34546 - protein, 9 aa, synthetic construct
GGSGDDIAY

SEQ ID NO: 34547 - protein, 9 aa, synthetic construct
GGSGDDHME

SEQ ID NO: 34548 - protein, 9 aa, synthetic construct
GGSGDDGIA

SEQ ID NO: 34549 - protein, 9 aa, synthetic construct
GGSGDDFIE

SEQ ID NO: 34550 - protein, 9 aa, synthetic construct
GGSGDDFIH

SEQ ID NO: 34551 - protein, 9 aa, synthetic construct
GGSGDDFIM

SEQ ID NO: 34552 - protein, 9 aa, synthetic construct
GGSGDDFLN

SEQ ID NO: 34553 - protein, 9 aa, synthetic construct
GGSGDDFLQ

SEQ ID NO: 34554 - protein, 9 aa, synthetic construct
GGSGDDFMD

SEQ ID NO: 34555 - protein, 9 aa, synthetic construct
GGSGDDFML

SEQ ID NO: 34556 - protein, 9 aa, synthetic construct
GGSGDDFMN

SEQ ID NO: 34557 - protein, 9 aa, synthetic construct
GGSGDDFMR

SEQ ID NO: 34558 - protein, 9 aa, synthetic construct
GGSGDDFVG

SEQ ID NO: 34559 - protein, 9 aa, synthetic construct
GGSGDDFVR

SEQ ID NO: 34560 - protein, 9 aa, synthetic construct
GGSGDDFVV

SEQ ID NO: 34561 - protein, 9 aa, synthetic construct
GGSGDDGFY

SEQ ID NO: 34562 - protein, 9 aa, synthetic construct
GGSGDDGID

SEQ ID NO: 34563 - protein, 9 aa, synthetic construct
GGSGDDHLN

SEQ ID NO: 34564 - protein, 9 aa, synthetic construct
GGSGDDGIW

SEQ ID NO: 34565 - protein, 9 aa, synthetic construct
GGSGDDGLA

SEQ ID NO: 34566 - protein, 9 aa, synthetic construct
GGSGDDGLG

SEQ ID NO: 34567 - protein, 9 aa, synthetic construct
GGSGDDGLK

SEQ ID NO: 34568 - protein, 9 aa, synthetic construct
GGSGDDGLN

SEQ ID NO: 34569 - protein, 9 aa, synthetic construct
GGSGDDGLV

SEQ ID NO: 34570 - protein, 9 aa, synthetic construct
GGSGDDGLY

SEQ ID NO: 34571 - protein, 9 aa, synthetic construct
GGSGDDHAF

SEQ ID NO: 34572 - protein, 9 aa, synthetic construct
GGSGDDHFI

SEQ ID NO: 34573 - protein, 9 aa, synthetic construct
GGSGDDHFN

SEQ ID NO: 34574 - protein, 9 aa, synthetic construct
GGSGDDHFY

SEQ ID NO: 34575 - protein, 9 aa, synthetic construct
GGSGDDHIV

SEQ ID NO: 34576 - protein, 9 aa, synthetic construct
GGSGDDHIY

SEQ ID NO: 34577 - protein, 9 aa, synthetic construct
GGSGDDLAE

SEQ ID NO: 34578 - protein, 9 aa, synthetic construct
GGSGDDLAL

SEQ ID NO: 34579 - protein, 9 aa, synthetic construct
GGSGDDLFD

SEQ ID NO: 34580 - protein, 9 aa, synthetic construct
GGSGDDQIF

SEQ ID NO: 34581 - protein, 9 aa, synthetic construct
GGSGDDNLG

SEQ ID NO: 34582 - protein, 9 aa, synthetic construct
GGSGDDNLI

SEQ ID NO: 34583 - protein, 9 aa, synthetic construct
GGSGDDNLV

SEQ ID NO: 34584 - protein, 9 aa, synthetic construct
GGSGDDNMR

SEQ ID NO: 34585 - protein, 9 aa, synthetic construct
GGSGDDNVF

SEQ ID NO: 34586 - protein, 9 aa, synthetic construct
GGSGDDNVK

SEQ ID NO: 34587 - protein, 9 aa, synthetic construct
GGSGDDQAN

SEQ ID NO: 34588 - protein, 9 aa, synthetic construct
GGSGDDQFF

SEQ ID NO: 34589 - protein, 9 aa, synthetic construct
GGSGDDQFI

SEQ ID NO: 34590 - protein, 9 aa, synthetic construct
GGSGDDQFN

SEQ ID NO: 34591 - protein, 9 aa, synthetic construct
GGSGDDQFV

SEQ ID NO: 34592 - protein, 9 aa, synthetic construct
GGSGDDQIA

SEQ ID NO: 34593 - protein, 9 aa, synthetic construct
GGSGDDQIE

SEQ ID NO: 34594 - protein, 9 aa, synthetic construct
GGSGDDQIR

SEQ ID NO: 34595 - protein, 9 aa, synthetic construct
GGSGDDNLA

SEQ ID NO: 34596 - protein, 9 aa, synthetic construct
GGSGDDQIS

SEQ ID NO: 34597 - protein, 9 aa, synthetic construct
GGSGDDQIY

SEQ ID NO: 34598 - protein, 9 aa, synthetic construct
GGSGDDQLG

SEQ ID NO: 34599 - protein, 9 aa, synthetic construct
GGSGDDQLQ

SEQ ID NO: 34600 - protein, 9 aa, synthetic construct
GGSGDDQLR

SEQ ID NO: 34601 - protein, 9 aa, synthetic construct
GGSGDDQVM

SEQ ID NO: 34602 - protein, 9 aa, synthetic construct
GGSGDDQVS

SEQ ID NO: 34603 - protein, 9 aa, synthetic construct
GGSGDDQVW

SEQ ID NO: 34604 - protein, 9 aa, synthetic construct
GGSGDDQYF

SEQ ID NO: 34605 - protein, 9 aa, synthetic construct
GGSGDDRAI

SEQ ID NO: 34606 - protein, 9 aa, synthetic construct
GGSGDDRAY

SEQ ID NO: 34607 - protein, 9 aa, synthetic construct
GGSGDDRFV

SEQ ID NO: 34608 - protein, 9 aa, synthetic construct
GGSGDDRFW

SEQ ID NO: 34609 - protein, 9 aa, synthetic construct
GGSGDDNLD

SEQ ID NO: 34610 - protein, 9 aa, synthetic construct
GGSGDDNIN

SEQ ID NO: 34611 - protein, 9 aa, synthetic construct
GGSGDDLFH

SEQ ID NO: 34612 - protein, 9 aa, synthetic construct
GGSGDDMAA

SEQ ID NO: 34613 - protein, 9 aa, synthetic construct
GGSGDDLFT

SEQ ID NO: 34614 - protein, 9 aa, synthetic construct
GGSGDDLFV

SEQ ID NO: 34615 - protein, 9 aa, synthetic construct
GGSGDDLIV

SEQ ID NO: 34616 - protein, 9 aa, synthetic construct
GGSGDDLLW

SEQ ID NO: 34617 - protein, 9 aa, synthetic construct
GGSGDDLMD

SEQ ID NO: 34618 - protein, 9 aa, synthetic construct
GGSGDDLMQ

SEQ ID NO: 34619 - protein, 9 aa, synthetic construct
GGSGDDLVA

SEQ ID NO: 34620 - protein, 9 aa, synthetic construct
GGSGDDLVG

SEQ ID NO: 34621 - protein, 9 aa, synthetic construct
GGSGDDLVI

SEQ ID NO: 34622 - protein, 9 aa, synthetic construct
GGSGDDLVK

SEQ ID NO: 34623 - protein, 9 aa, synthetic construct
GGSGDDLVL

SEQ ID NO: 34624 - protein, 9 aa, synthetic construct
GGSGDDLVT

SEQ ID NO: 34625 - protein, 9 aa, synthetic construct
GGSGDDLYR

SEQ ID NO: 34626 - protein, 9 aa, synthetic construct
GGSGDDMAY

SEQ ID NO: 34627 - protein, 9 aa, synthetic construct
GGSGDDNIK

SEQ ID NO: 34628 - protein, 9 aa, synthetic construct
GGSGDDMIA

SEQ ID NO: 34629 - protein, 9 aa, synthetic construct
GGSGDDMIE

SEQ ID NO: 34630 - protein, 9 aa, synthetic construct
GGSGDDMIF

SEQ ID NO: 34631 - protein, 9 aa, synthetic construct
GGSGDDMIS

SEQ ID NO: 34632 - protein, 9 aa, synthetic construct
GGSGDDMIT

SEQ ID NO: 34633 - protein, 9 aa, synthetic construct
GGSGDDMIW

SEQ ID NO: 34634 - protein, 9 aa, synthetic construct
GGSGDDMIY

SEQ ID NO: 34635 - protein, 9 aa, synthetic construct
GGSGDDMLQ

SEQ ID NO: 34636 - protein, 9 aa, synthetic construct
GGSGDDMLY

SEQ ID NO: 34637 - protein, 9 aa, synthetic construct
GGSGDDMVF

SEQ ID NO: 34638 - protein, 9 aa, synthetic construct
GGSGDDMVI

SEQ ID NO: 34639 - protein, 9 aa, synthetic construct
GGSGDDNFL

SEQ ID NO: 34640 - protein, 9 aa, synthetic construct
GGSGDDNFT

SEQ ID NO: 34641 - protein, 9 aa, synthetic construct
GGSGADFLW

SEQ ID NO: 34642 - protein, 9 aa, synthetic construct
GGSGADFLQ

SEQ ID NO: 34643 - protein, 9 aa, synthetic construct
GGSGRDLLH

SEQ ID NO: 34644 - protein, 9 aa, synthetic construct
GGRGQDNLQ

SEQ ID NO: 34645 - protein, 9 aa, synthetic construct
GGRGNDWLQ

SEQ ID NO: 34646 - protein, 9 aa, synthetic construct
GGRGNDWLT

SEQ ID NO: 34647 - protein, 9 aa, synthetic construct
GGRGNDYAW

SEQ ID NO: 34648 - protein, 9 aa, synthetic construct
GGRGNDYID

SEQ ID NO: 34649 - protein, 9 aa, synthetic construct
GGRGNDYLV

SEQ ID NO: 34650 - protein, 9 aa, synthetic construct
GGRGNDYVD

SEQ ID NO: 34651 - protein, 9 aa, synthetic construct
GGRGNDYVH

SEQ ID NO: 34652 - protein, 9 aa, synthetic construct
GGRGPDDLY

SEQ ID NO: 34653 - protein, 9 aa, synthetic construct
GGRGPDEIR

SEQ ID NO: 34654 - protein, 9 aa, synthetic construct
GGRGPDIFQ

SEQ ID NO: 34655 - protein, 9 aa, synthetic construct
GGRGPDMFV

SEQ ID NO: 34656 - protein, 9 aa, synthetic construct
GGRGPDRLL

SEQ ID NO: 34657 - protein, 9 aa, synthetic construct
GGRGPDRLN

SEQ ID NO: 34658 - protein, 9 aa, synthetic construct
GGRGPDRLS

SEQ ID NO: 34659 - protein, 9 aa, synthetic construct
GGRGPDSIY

SEQ ID NO: 34660 - protein, 9 aa, synthetic construct
GGRGPDTFF

SEQ ID NO: 34661 - protein, 9 aa, synthetic construct
GGRGPDVLC

SEQ ID NO: 34662 - protein, 9 aa, synthetic construct
GGRGPDVLT

SEQ ID NO: 34663 - protein, 9 aa, synthetic construct
GGRGQDDLD

SEQ ID NO: 34664 - protein, 9 aa, synthetic construct
GGRGQDELQ

SEQ ID NO: 34665 - protein, 9 aa, synthetic construct
GGRGQDFFF

SEQ ID NO: 34666 - protein, 9 aa, synthetic construct
GGRGQDFLF

SEQ ID NO: 34667 - protein, 9 aa, synthetic construct
GGRGQDFLN

SEQ ID NO: 34668 - protein, 9 aa, synthetic construct
GGRGQDHLY

SEQ ID NO: 34669 - protein, 9 aa, synthetic construct
GGRGQDIID

SEQ ID NO: 34670 - protein, 9 aa, synthetic construct
GGRGQDILR

SEQ ID NO: 34671 - protein, 9 aa, synthetic construct
GGRGQDKLI

SEQ ID NO: 34672 - protein, 9 aa, synthetic construct
GGRGQDLLI

SEQ ID NO: 34673 - protein, 9 aa, synthetic construct
GGRGQDLLN

SEQ ID NO: 34674 - protein, 9 aa, synthetic construct
GGRGNDWLF

SEQ ID NO: 34675 - protein, 9 aa, synthetic construct
GGRGNDWLE

SEQ ID NO: 34676 - protein, 9 aa, synthetic construct
GGRGNDWIN

SEQ ID NO: 34677 - protein, 9 aa, synthetic construct
GGRGNDTYA

SEQ ID NO: 34678 - protein, 9 aa, synthetic construct
GGRGNDTAS

SEQ ID NO: 34679 - protein, 9 aa, synthetic construct
GGRGNDTAT

SEQ ID NO: 34680 - protein, 9 aa, synthetic construct
GGRGNDTAV

SEQ ID NO: 34681 - protein, 9 aa, synthetic construct
GGRGNDTFD

SEQ ID NO: 34682 - protein, 9 aa, synthetic construct
GGRGNDTFI

SEQ ID NO: 34683 - protein, 9 aa, synthetic construct
GGRGNDTIS

SEQ ID NO: 34684 - protein, 9 aa, synthetic construct
GGRGNDTIT

SEQ ID NO: 34685 - protein, 9 aa, synthetic construct
GGRGNDTIW

SEQ ID NO: 34686 - protein, 9 aa, synthetic construct
GGRGNDTMD

SEQ ID NO: 34687 - protein, 9 aa, synthetic construct
GGRGNDTMN

SEQ ID NO: 34688 - protein, 9 aa, synthetic construct
GGRGNDTVF

SEQ ID NO: 34689 - protein, 9 aa, synthetic construct
GGRGNDTVG

SEQ ID NO: 34690 - protein, 9 aa, synthetic construct
GGRGNDTVS

SEQ ID NO: 34691 - protein, 9 aa, synthetic construct
GGRGNDTYK

SEQ ID NO: 34692 - protein, 9 aa, synthetic construct
GGRGNDWIE

SEQ ID NO: 34693 - protein, 9 aa, synthetic construct
GGRGNDTYT

SEQ ID NO: 34694 - protein, 9 aa, synthetic construct
GGRGNDVAY

SEQ ID NO: 34695 - protein, 9 aa, synthetic construct
GGRGNDVFE

SEQ ID NO: 34696 - protein, 9 aa, synthetic construct
GGRGNDVIH

SEQ ID NO: 34697 - protein, 9 aa, synthetic construct
GGRGNDVIL

SEQ ID NO: 34698 - protein, 9 aa, synthetic construct
GGRGNDVIS

SEQ ID NO: 34699 - protein, 9 aa, synthetic construct
GGRGNDVIV

SEQ ID NO: 34700 - protein, 9 aa, synthetic construct
GGRGNDVIW

SEQ ID NO: 34701 - protein, 9 aa, synthetic construct
GGRGNDVLG

SEQ ID NO: 34702 - protein, 9 aa, synthetic construct
GGRGNDVLW

SEQ ID NO: 34703 - protein, 9 aa, synthetic construct
GGRGNDVMN

SEQ ID NO: 34704 - protein, 9 aa, synthetic construct
GGRGNDVMS

SEQ ID NO: 34705 - protein, 9 aa, synthetic construct
GGRGNDWID

SEQ ID NO: 34706 - protein, 9 aa, synthetic construct
GGRGQDLMT

SEQ ID NO: 34707 - protein, 9 aa, synthetic construct
GGRGQDRLS

SEQ ID NO: 34708 - protein, 9 aa, synthetic construct
GGRGRDRLY

SEQ ID NO: 34709 - protein, 9 aa, synthetic construct
GGRGQDRLT

SEQ ID NO: 34710 - protein, 9 aa, synthetic construct
GGRGRDKLI

SEQ ID NO: 34711 - protein, 9 aa, synthetic construct
GGRGRDKLK

SEQ ID NO: 34712 - protein, 9 aa, synthetic construct
GGRGRDKLM

SEQ ID NO: 34713 - protein, 9 aa, synthetic construct
GGRGRDKLS

SEQ ID NO: 34714 - protein, 9 aa, synthetic construct
GGRGRDKLV

SEQ ID NO: 34715 - protein, 9 aa, synthetic construct
GGRGRDLAD

SEQ ID NO: 34716 - protein, 9 aa, synthetic construct
GGRGRDLFI

SEQ ID NO: 34717 - protein, 9 aa, synthetic construct
GGRGRDLLF

SEQ ID NO: 34718 - protein, 9 aa, synthetic construct
GGRGRDLLI

SEQ ID NO: 34719 - protein, 9 aa, synthetic construct
GGRGRDLLL

SEQ ID NO: 34720 - protein, 9 aa, synthetic construct
GGRGRDLLW

SEQ ID NO: 34721 - protein, 9 aa, synthetic construct
GGRGRDLVD

SEQ ID NO: 34722 - protein, 9 aa, synthetic construct
GGRGRDNFW

SEQ ID NO: 34723 - protein, 9 aa, synthetic construct
GGRGRDNIF

SEQ ID NO: 34724 - protein, 9 aa, synthetic construct
GGRGRDNLK

SEQ ID NO: 34725 - protein, 9 aa, synthetic construct
GGRGRDNLL

SEQ ID NO: 34726 - protein, 9 aa, synthetic construct
GGRGRDNLR

SEQ ID NO: 34727 - protein, 9 aa, synthetic construct
GGRGRDNVW

SEQ ID NO: 34728 - protein, 9 aa, synthetic construct
GGRGRDQLH

SEQ ID NO: 34729 - protein, 9 aa, synthetic construct
GGRGRDQLS

SEQ ID NO: 34730 - protein, 9 aa, synthetic construct
GGRGRDQLY

SEQ ID NO: 34731 - protein, 9 aa, synthetic construct
GGRGRDQMT

SEQ ID NO: 34732 - protein, 9 aa, synthetic construct
GGRGRDRFV

SEQ ID NO: 34733 - protein, 9 aa, synthetic construct
GGRGRDRID

SEQ ID NO: 34734 - protein, 9 aa, synthetic construct
GGRGRDRIE

SEQ ID NO: 34735 - protein, 9 aa, synthetic construct
GGRGRDRIF

SEQ ID NO: 34736 - protein, 9 aa, synthetic construct
GGRGRDRIH

SEQ ID NO: 34737 - protein, 9 aa, synthetic construct
GGRGRDRLL

SEQ ID NO: 34738 - protein, 9 aa, synthetic construct
GGRGRDRLR

SEQ ID NO: 34739 - protein, 9 aa, synthetic construct
GGRGRDKIY

SEQ ID NO: 34740 - protein, 9 aa, synthetic construct
GGRGRDILK

SEQ ID NO: 34741 - protein, 9 aa, synthetic construct
GGRGRDILF

SEQ ID NO: 34742 - protein, 9 aa, synthetic construct
GGRGQDYIN

SEQ ID NO: 34743 - protein, 9 aa, synthetic construct
GGRGQDRLY

SEQ ID NO: 34744 - protein, 9 aa, synthetic construct
GGRGQDSLA

SEQ ID NO: 34745 - protein, 9 aa, synthetic construct
GGRGQDTLD

SEQ ID NO: 34746 - protein, 9 aa, synthetic construct
GGRGQDTLL

SEQ ID NO: 34747 - protein, 9 aa, synthetic construct
GGRGQDTLS

SEQ ID NO: 34748 - protein, 9 aa, synthetic construct
GGRGQDTLY

SEQ ID NO: 34749 - protein, 9 aa, synthetic construct
GGRGQDVAF

SEQ ID NO: 34750 - protein, 9 aa, synthetic construct
GGRGQDVFR

SEQ ID NO: 34751 - protein, 9 aa, synthetic construct
GGRGQDVFV

SEQ ID NO: 34752 - protein, 9 aa, synthetic construct
GGRGQDVIT

SEQ ID NO: 34753 - protein, 9 aa, synthetic construct
GGRGQDVLN

SEQ ID NO: 34754 - protein, 9 aa, synthetic construct
GGRGQDVMT

SEQ ID NO: 34755 - protein, 9 aa, synthetic construct
GGRGQDWLE

SEQ ID NO: 34756 - protein, 9 aa, synthetic construct
GGRGQDYLY

SEQ ID NO: 34757 - protein, 9 aa, synthetic construct
GGRGRDFMF

SEQ ID NO: 34758 - protein, 9 aa, synthetic construct
GGRGRDAID

SEQ ID NO: 34759 - protein, 9 aa, synthetic construct
GGRGRDALE

SEQ ID NO: 34760 - protein, 9 aa, synthetic construct
GGRGRDALN

SEQ ID NO: 34761 - protein, 9 aa, synthetic construct
GGRGRDALR

SEQ ID NO: 34762 - protein, 9 aa, synthetic construct
GGRGRDDIH

SEQ ID NO: 34763 - protein, 9 aa, synthetic construct
GGRGRDDLA

SEQ ID NO: 34764 - protein, 9 aa, synthetic construct
GGRGRDDLF

SEQ ID NO: 34765 - protein, 9 aa, synthetic construct
GGRGRDDMD

SEQ ID NO: 34766 - protein, 9 aa, synthetic construct
GGRGRDEIF

SEQ ID NO: 34767 - protein, 9 aa, synthetic construct
GGRGRDELS

SEQ ID NO: 34768 - protein, 9 aa, synthetic construct
GGRGRDELT

SEQ ID NO: 34769 - protein, 9 aa, synthetic construct
GGRGRDFLF

SEQ ID NO: 34770 - protein, 9 aa, synthetic construct
GGRGRDFLL

SEQ ID NO: 34771 - protein, 9 aa, synthetic construct
GGRGNDTAF

SEQ ID NO: 34772 - protein, 9 aa, synthetic construct
GGRGNDSYY

SEQ ID NO: 34773 - protein, 9 aa, synthetic construct
GGRGNDSVV

SEQ ID NO: 34774 - protein, 9 aa, synthetic construct
GGRGNDSVS

SEQ ID NO: 34775 - protein, 9 aa, synthetic construct
GGRGNDFLH

SEQ ID NO: 34776 - protein, 9 aa, synthetic construct
GGRGNDFLL

SEQ ID NO: 34777 - protein, 9 aa, synthetic construct
GGRGNDGLT

SEQ ID NO: 34778 - protein, 9 aa, synthetic construct
GGRGNDGLV

SEQ ID NO: 34779 - protein, 9 aa, synthetic construct
GGRGNDHFE

SEQ ID NO: 34780 - protein, 9 aa, synthetic construct
GGRGNDHIS

SEQ ID NO: 34781 - protein, 9 aa, synthetic construct
GGRGNDHIY

SEQ ID NO: 34782 - protein, 9 aa, synthetic construct
GGRGNDHLE

SEQ ID NO: 34783 - protein, 9 aa, synthetic construct
GGRGNDHLF

SEQ ID NO: 34784 - protein, 9 aa, synthetic construct
GGRGNDHLS

SEQ ID NO: 34785 - protein, 9 aa, synthetic construct
GGRGNDHLT

SEQ ID NO: 34786 - protein, 9 aa, synthetic construct
GGRGNDIFH

SEQ ID NO: 34787 - protein, 9 aa, synthetic construct
GGRGNDIFI

SEQ ID NO: 34788 - protein, 9 aa, synthetic construct
GGRGNDIIF

SEQ ID NO: 34789 - protein, 9 aa, synthetic construct
GGRGNDIIG

SEQ ID NO: 34790 - protein, 9 aa, synthetic construct
GGRGNDIIL

SEQ ID NO: 34791 - protein, 9 aa, synthetic construct
GGRGNDIIQ

SEQ ID NO: 34792 - protein, 9 aa, synthetic construct
GGRGNDIIR

SEQ ID NO: 34793 - protein, 9 aa, synthetic construct
GGRGNDIIV

SEQ ID NO: 34794 - protein, 9 aa, synthetic construct
GGRGNDIIY

SEQ ID NO: 34795 - protein, 9 aa, synthetic construct
GGRGNDILH

SEQ ID NO: 34796 - protein, 9 aa, synthetic construct
GGRGNDILM

SEQ ID NO: 34797 - protein, 9 aa, synthetic construct
GGRGNDIMD

SEQ ID NO: 34798 - protein, 9 aa, synthetic construct
GGRGNDIMY

SEQ ID NO: 34799 - protein, 9 aa, synthetic construct
GGRGNDIYV

SEQ ID NO: 34800 - protein, 9 aa, synthetic construct
GGRGNDKIG

SEQ ID NO: 34801 - protein, 9 aa, synthetic construct
GGRGNDKIS

SEQ ID NO: 34802 - protein, 9 aa, synthetic construct
GGRGNDKLA

SEQ ID NO: 34803 - protein, 9 aa, synthetic construct
GGRGNDKLT

SEQ ID NO: 34804 - protein, 9 aa, synthetic construct
GGRGNDFIY

SEQ ID NO: 34805 - protein, 9 aa, synthetic construct
GGRGNDFIF

SEQ ID NO: 34806 - protein, 9 aa, synthetic construct
GGRGNDEVY

SEQ ID NO: 34807 - protein, 9 aa, synthetic construct
GGRGNDAVM

SEQ ID NO: 34808 - protein, 9 aa, synthetic construct
GGRGNDAFY

SEQ ID NO: 34809 - protein, 9 aa, synthetic construct
GGRGNDAIA

SEQ ID NO: 34810 - protein, 9 aa, synthetic construct
GGRGNDAID

SEQ ID NO: 34811 - protein, 9 aa, synthetic construct
GGRGNDAIW

SEQ ID NO: 34812 - protein, 9 aa, synthetic construct
GGRGNDALA

SEQ ID NO: 34813 - protein, 9 aa, synthetic construct
GGRGNDALF

SEQ ID NO: 34814 - protein, 9 aa, synthetic construct
GGRGNDALI

SEQ ID NO: 34815 - protein, 9 aa, synthetic construct
GGRGNDALK

SEQ ID NO: 34816 - protein, 9 aa, synthetic construct
GGRGNDALN

SEQ ID NO: 34817 - protein, 9 aa, synthetic construct
GGRGNDALT

SEQ ID NO: 34818 - protein, 9 aa, synthetic construct
GGRGNDALV

SEQ ID NO: 34819 - protein, 9 aa, synthetic construct
GGRGNDAMA

SEQ ID NO: 34820 - protein, 9 aa, synthetic construct
GGRGNDAMI

SEQ ID NO: 34821 - protein, 9 aa, synthetic construct
GGRGNDDIF

SEQ ID NO: 34822 - protein, 9 aa, synthetic construct
GGRGNDELT

SEQ ID NO: 34823 - protein, 9 aa, synthetic construct
GGRGNDDIL

SEQ ID NO: 34824 - protein, 9 aa, synthetic construct
GGRGNDDLD

SEQ ID NO: 34825 - protein, 9 aa, synthetic construct
GGRGNDDLG

SEQ ID NO: 34826 - protein, 9 aa, synthetic construct
GGRGNDDLL

SEQ ID NO: 34827 - protein, 9 aa, synthetic construct
GGRGNDDLQ

SEQ ID NO: 34828 - protein, 9 aa, synthetic construct
GGRGNDDLY

SEQ ID NO: 34829 - protein, 9 aa, synthetic construct
GGRGNDEAY

SEQ ID NO: 34830 - protein, 9 aa, synthetic construct
GGRGNDEIE

SEQ ID NO: 34831 - protein, 9 aa, synthetic construct
GGRGNDEIG

SEQ ID NO: 34832 - protein, 9 aa, synthetic construct
GGRGNDEIL

SEQ ID NO: 34833 - protein, 9 aa, synthetic construct
GGRGNDEIR

SEQ ID NO: 34834 - protein, 9 aa, synthetic construct
GGRGNDEIT

SEQ ID NO: 34835 - protein, 9 aa, synthetic construct
GGRGNDELS

SEQ ID NO: 34836 - protein, 9 aa, synthetic construct
GGRGNDKLY

SEQ ID NO: 34837 - protein, 9 aa, synthetic construct
GGRGNDLAF

SEQ ID NO: 34838 - protein, 9 aa, synthetic construct
GGRGNDLAL

SEQ ID NO: 34839 - protein, 9 aa, synthetic construct
GGRGNDRVV

SEQ ID NO: 34840 - protein, 9 aa, synthetic construct
GGRGNDQMR

SEQ ID NO: 34841 - protein, 9 aa, synthetic construct
GGRGNDQMS

SEQ ID NO: 34842 - protein, 9 aa, synthetic construct
GGRGNDRAD

SEQ ID NO: 34843 - protein, 9 aa, synthetic construct
GGRGNDRAW

SEQ ID NO: 34844 - protein, 9 aa, synthetic construct
GGRGNDRFL

SEQ ID NO: 34845 - protein, 9 aa, synthetic construct
GGRGNDRFY

SEQ ID NO: 34846 - protein, 9 aa, synthetic construct
GGRGNDRIE

SEQ ID NO: 34847 - protein, 9 aa, synthetic construct
GGRGNDRIK

SEQ ID NO: 34848 - protein, 9 aa, synthetic construct
GGRGNDRIS

SEQ ID NO: 34849 - protein, 9 aa, synthetic construct
GGRGNDRIV

SEQ ID NO: 34850 - protein, 9 aa, synthetic construct
GGRGNDRLG

SEQ ID NO: 34851 - protein, 9 aa, synthetic construct
GGRGNDRMS

SEQ ID NO: 34852 - protein, 9 aa, synthetic construct
GGRGNDRMV

SEQ ID NO: 34853 - protein, 9 aa, synthetic construct
GGRGNDRYL

SEQ ID NO: 34854 - protein, 9 aa, synthetic construct
GGRGNDQLT

SEQ ID NO: 34855 - protein, 9 aa, synthetic construct
GGRGNDRYV

SEQ ID NO: 34856 - protein, 9 aa, synthetic construct
GGRGNDSAT

SEQ ID NO: 34857 - protein, 9 aa, synthetic construct
GGRGNDSFR

SEQ ID NO: 34858 - protein, 9 aa, synthetic construct
GGRGNDSIA

SEQ ID NO: 34859 - protein, 9 aa, synthetic construct
GGRGNDSID

SEQ ID NO: 34860 - protein, 9 aa, synthetic construct
GGRGNDSIG

SEQ ID NO: 34861 - protein, 9 aa, synthetic construct
GGRGNDSIL

SEQ ID NO: 34862 - protein, 9 aa, synthetic construct
GGRGNDSIV

SEQ ID NO: 34863 - protein, 9 aa, synthetic construct
GGRGNDSLF

SEQ ID NO: 34864 - protein, 9 aa, synthetic construct
GGRGNDSLL

SEQ ID NO: 34865 - protein, 9 aa, synthetic construct
GGRGNDSLW

SEQ ID NO: 34866 - protein, 9 aa, synthetic construct
GGRGNDSMS

SEQ ID NO: 34867 - protein, 9 aa, synthetic construct
GGRGNDSMT

SEQ ID NO: 34868 - protein, 9 aa, synthetic construct
GGRGNDQLV

SEQ ID NO: 34869 - protein, 9 aa, synthetic construct
GGRGNDQLN

SEQ ID NO: 34870 - protein, 9 aa, synthetic construct
GGRGNDLID

SEQ ID NO: 34871 - protein, 9 aa, synthetic construct
GGRGNDNIE

SEQ ID NO: 34872 - protein, 9 aa, synthetic construct
GGRGNDLIE

SEQ ID NO: 34873 - protein, 9 aa, synthetic construct
GGRGNDLIF

SEQ ID NO: 34874 - protein, 9 aa, synthetic construct
GGRGNDLIH

SEQ ID NO: 34875 - protein, 9 aa, synthetic construct
GGRGNDLIT

SEQ ID NO: 34876 - protein, 9 aa, synthetic construct
GGRGNDLLM

SEQ ID NO: 34877 - protein, 9 aa, synthetic construct
GGRGNDLLN

SEQ ID NO: 34878 - protein, 9 aa, synthetic construct
GGRGNDLLW

SEQ ID NO: 34879 - protein, 9 aa, synthetic construct
GGRGNDLMG

SEQ ID NO: 34880 - protein, 9 aa, synthetic construct
GGRGNDLVF

SEQ ID NO: 34881 - protein, 9 aa, synthetic construct
GGRGNDLVV

SEQ ID NO: 34882 - protein, 9 aa, synthetic construct
GGRGNDLYR

SEQ ID NO: 34883 - protein, 9 aa, synthetic construct
GGRGNDLYY

SEQ ID NO: 34884 - protein, 9 aa, synthetic construct
GGRGNDMLH

SEQ ID NO: 34885 - protein, 9 aa, synthetic construct
GGRGNDNIF

SEQ ID NO: 34886 - protein, 9 aa, synthetic construct
GGRGNDQLG

SEQ ID NO: 34887 - protein, 9 aa, synthetic construct
GGRGNDNIS

SEQ ID NO: 34888 - protein, 9 aa, synthetic construct
GGRGNDNIT

SEQ ID NO: 34889 - protein, 9 aa, synthetic construct
GGRGNDNLD

SEQ ID NO: 34890 - protein, 9 aa, synthetic construct
GGRGNDNLG

SEQ ID NO: 34891 - protein, 9 aa, synthetic construct
GGRGNDNLK

SEQ ID NO: 34892 - protein, 9 aa, synthetic construct
GGRGNDNLN

SEQ ID NO: 34893 - protein, 9 aa, synthetic construct
GGRGNDNLY

SEQ ID NO: 34894 - protein, 9 aa, synthetic construct
GGRGNDNVS

SEQ ID NO: 34895 - protein, 9 aa, synthetic construct
GGRGNDNYV

SEQ ID NO: 34896 - protein, 9 aa, synthetic construct
GGRGNDQFF

SEQ ID NO: 34897 - protein, 9 aa, synthetic construct
GGRGNDQID

SEQ ID NO: 34898 - protein, 9 aa, synthetic construct
GGRGNDQIN

SEQ ID NO: 34899 - protein, 9 aa, synthetic construct
GGRGNDQIW

SEQ ID NO: 34900 - protein, 9 aa, synthetic construct
GGRGRDRLT

SEQ ID NO: 34901 - protein, 9 aa, synthetic construct
GGRGRDRMV

SEQ ID NO: 34902 - protein, 9 aa, synthetic construct
GGSGADFLK

SEQ ID NO: 34903 - protein, 9 aa, synthetic construct
GGRGVDTLA

SEQ ID NO: 34904 - protein, 9 aa, synthetic construct
GGRGTDVLK

SEQ ID NO: 34905 - protein, 9 aa, synthetic construct
GGRGTDVLT

SEQ ID NO: 34906 - protein, 9 aa, synthetic construct
GGRGTDWLM

SEQ ID NO: 34907 - protein, 9 aa, synthetic construct
GGRGVDAFH

SEQ ID NO: 34908 - protein, 9 aa, synthetic construct
GGRGVDAFV

SEQ ID NO: 34909 - protein, 9 aa, synthetic construct
GGRGVDALI

SEQ ID NO: 34910 - protein, 9 aa, synthetic construct
GGRGVDEVY

SEQ ID NO: 34911 - protein, 9 aa, synthetic construct
GGRGVDHVD

SEQ ID NO: 34912 - protein, 9 aa, synthetic construct
GGRGVDIFR

SEQ ID NO: 34913 - protein, 9 aa, synthetic construct
GGRGVDILG

SEQ ID NO: 34914 - protein, 9 aa, synthetic construct
GGRGVDILK

SEQ ID NO: 34915 - protein, 9 aa, synthetic construct
GGRGVDILR

SEQ ID NO: 34916 - protein, 9 aa, synthetic construct
GGRGVDILS

SEQ ID NO: 34917 - protein, 9 aa, synthetic construct
GGRGVDKLY

SEQ ID NO: 34918 - protein, 9 aa, synthetic construct
GGRGVDLLT

SEQ ID NO: 34919 - protein, 9 aa, synthetic construct
GGRGVDLLV

SEQ ID NO: 34920 - protein, 9 aa, synthetic construct
GGRGVDMLT

SEQ ID NO: 34921 - protein, 9 aa, synthetic construct
GGRGVDQLT

SEQ ID NO: 34922 - protein, 9 aa, synthetic construct
GGRGVDRLE

SEQ ID NO: 34923 - protein, 9 aa, synthetic construct
GGRGVDRLT

SEQ ID NO: 34924 - protein, 9 aa, synthetic construct
GGRGVDRLV

SEQ ID NO: 34925 - protein, 9 aa, synthetic construct
GGRGVDRME

SEQ ID NO: 34926 - protein, 9 aa, synthetic construct
GGRGVDSLT

SEQ ID NO: 34927 - protein, 9 aa, synthetic construct
GGRGVDTAL

SEQ ID NO: 34928 - protein, 9 aa, synthetic construct
GGRGVDTAS

SEQ ID NO: 34929 - protein, 9 aa, synthetic construct
GGRGVDTFR

SEQ ID NO: 34930 - protein, 9 aa, synthetic construct
GGRGVDTFV

SEQ ID NO: 34931 - protein, 9 aa, synthetic construct
GGRGVDTIN

SEQ ID NO: 34932 - protein, 9 aa, synthetic construct
GGRGVDTIS

SEQ ID NO: 34933 - protein, 9 aa, synthetic construct
GGRGTDVAM

SEQ ID NO: 34934 - protein, 9 aa, synthetic construct
GGRGTDTML

SEQ ID NO: 34935 - protein, 9 aa, synthetic construct
GGRGTDTLR

SEQ ID NO: 34936 - protein, 9 aa, synthetic construct
GGRGTDLLT

SEQ ID NO: 34937 - protein, 9 aa, synthetic construct
GGRGSDYVM

SEQ ID NO: 34938 - protein, 9 aa, synthetic construct
GGRGTDAID

SEQ ID NO: 34939 - protein, 9 aa, synthetic construct
GGRGTDAIF

SEQ ID NO: 34940 - protein, 9 aa, synthetic construct
GGRGTDALY

SEQ ID NO: 34941 - protein, 9 aa, synthetic construct
GGRGTDDLL

SEQ ID NO: 34942 - protein, 9 aa, synthetic construct
GGRGTDFIE

SEQ ID NO: 34943 - protein, 9 aa, synthetic construct
GGRGTDFLA

SEQ ID NO: 34944 - protein, 9 aa, synthetic construct
GGRGTDIFE

SEQ ID NO: 34945 - protein, 9 aa, synthetic construct
GGRGTDIFL

SEQ ID NO: 34946 - protein, 9 aa, synthetic construct
GGRGTDIFV

SEQ ID NO: 34947 - protein, 9 aa, synthetic construct
GGRGTDILW

SEQ ID NO: 34948 - protein, 9 aa, synthetic construct
GGRGTDIMF

SEQ ID NO: 34949 - protein, 9 aa, synthetic construct
GGRGTDLIG

SEQ ID NO: 34950 - protein, 9 aa, synthetic construct
GGRGTDLLY

SEQ ID NO: 34951 - protein, 9 aa, synthetic construct
GGRGTDTAD

SEQ ID NO: 34952 - protein, 9 aa, synthetic construct
GGRGTDLML

SEQ ID NO: 34953 - protein, 9 aa, synthetic construct
GGRGTDMLL

SEQ ID NO: 34954 - protein, 9 aa, synthetic construct
GGRGTDMLR

SEQ ID NO: 34955 - protein, 9 aa, synthetic construct
GGRGTDQLF

SEQ ID NO: 34956 - protein, 9 aa, synthetic construct
GGRGTDQLY

SEQ ID NO: 34957 - protein, 9 aa, synthetic construct
GGRGTDRAI

SEQ ID NO: 34958 - protein, 9 aa, synthetic construct
GGRGTDRLI

SEQ ID NO: 34959 - protein, 9 aa, synthetic construct
GGRGTDRLR

SEQ ID NO: 34960 - protein, 9 aa, synthetic construct
GGRGTDRLS

SEQ ID NO: 34961 - protein, 9 aa, synthetic construct
GGRGTDSLN

SEQ ID NO: 34962 - protein, 9 aa, synthetic construct
GGRGTDSLS

SEQ ID NO: 34963 - protein, 9 aa, synthetic construct
GGRGTDSLT

SEQ ID NO: 34964 - protein, 9 aa, synthetic construct
GGRGTDSYV

SEQ ID NO: 34965 - protein, 9 aa, synthetic construct
GGRGVDTIV

SEQ ID NO: 34966 - protein, 9 aa, synthetic construct
GGRGVDTLF

SEQ ID NO: 34967 - protein, 9 aa, synthetic construct
GGRGRDRVF

SEQ ID NO: 34968 - protein, 9 aa, synthetic construct
GGRGVDTLT

SEQ ID NO: 34969 - protein, 9 aa, synthetic construct
GGSGADDLI

SEQ ID NO: 34970 - protein, 9 aa, synthetic construct
GGSGADDLN

SEQ ID NO: 34971 - protein, 9 aa, synthetic construct
GGSGADDMA

SEQ ID NO: 34972 - protein, 9 aa, synthetic construct
GGSGADDMF

SEQ ID NO: 34973 - protein, 9 aa, synthetic construct
GGSGADDMQ

SEQ ID NO: 34974 - protein, 9 aa, synthetic construct
GGSGADDYI

SEQ ID NO: 34975 - protein, 9 aa, synthetic construct
GGSGADEFE

SEQ ID NO: 34976 - protein, 9 aa, synthetic construct
GGSGADEFF

SEQ ID NO: 34977 - protein, 9 aa, synthetic construct
GGSGADEFS

SEQ ID NO: 34978 - protein, 9 aa, synthetic construct
GGSGADEIF

SEQ ID NO: 34979 - protein, 9 aa, synthetic construct
GGSGADEIT

SEQ ID NO: 34980 - protein, 9 aa, synthetic construct
GGSGADEIW

SEQ ID NO: 34981 - protein, 9 aa, synthetic construct
GGSGADELA

SEQ ID NO: 34982 - protein, 9 aa, synthetic construct
GGSGADELF

SEQ ID NO: 34983 - protein, 9 aa, synthetic construct
GGSGADELI

SEQ ID NO: 34984 - protein, 9 aa, synthetic construct
GGSGADELN

SEQ ID NO: 34985 - protein, 9 aa, synthetic construct
GGSGADELT

SEQ ID NO: 34986 - protein, 9 aa, synthetic construct
GGSGADELV

SEQ ID NO: 34987 - protein, 9 aa, synthetic construct
GGSGADELW

SEQ ID NO: 34988 - protein, 9 aa, synthetic construct
GGSGADEMG

SEQ ID NO: 34989 - protein, 9 aa, synthetic construct
GGSGADEML

SEQ ID NO: 34990 - protein, 9 aa, synthetic construct
GGSGADEMV

SEQ ID NO: 34991 - protein, 9 aa, synthetic construct
GGSGADEMW

SEQ ID NO: 34992 - protein, 9 aa, synthetic construct
GGSGADEVD

SEQ ID NO: 34993 - protein, 9 aa, synthetic construct
GGSGADEVS

SEQ ID NO: 34994 - protein, 9 aa, synthetic construct
GGSGADFAR

SEQ ID NO: 34995 - protein, 9 aa, synthetic construct
GGSGADFIF

SEQ ID NO: 34996 - protein, 9 aa, synthetic construct
GGSGADFIR

SEQ ID NO: 34997 - protein, 9 aa, synthetic construct
GGSGADFIY

SEQ ID NO: 34998 - protein, 9 aa, synthetic construct
GGSGADDLH

SEQ ID NO: 34999 - protein, 9 aa, synthetic construct
GGSGADDIR

SEQ ID NO: 35000 - protein, 9 aa, synthetic construct
GGSGADDIN

SEQ ID NO: 35001 - protein, 9 aa, synthetic construct
GGRGYDQFH

SEQ ID NO: 35002 - protein, 9 aa, synthetic construct
GGRGVDTMT

SEQ ID NO: 35003 - protein, 9 aa, synthetic construct
GGRGVDTVV

SEQ ID NO: 35004 - protein, 9 aa, synthetic construct
GGRGVDVLF

SEQ ID NO: 35005 - protein, 9 aa, synthetic construct
GGRGVDWMT

SEQ ID NO: 35006 - protein, 9 aa, synthetic construct
GGRGVDWVN

SEQ ID NO: 35007 - protein, 9 aa, synthetic construct
GGRGWDFLF

SEQ ID NO: 35008 - protein, 9 aa, synthetic construct
GGRGWDILD

SEQ ID NO: 35009 - protein, 9 aa, synthetic construct
GGRGWDLMD

SEQ ID NO: 35010 - protein, 9 aa, synthetic construct
GGRGWDRLE

SEQ ID NO: 35011 - protein, 9 aa, synthetic construct
GGRGWDTAL

SEQ ID NO: 35012 - protein, 9 aa, synthetic construct
GGRGWDVLE

SEQ ID NO: 35013 - protein, 9 aa, synthetic construct
GGRGYDFVD

SEQ ID NO: 35014 - protein, 9 aa, synthetic construct
GGRGYDLFT

SEQ ID NO: 35015 - protein, 9 aa, synthetic construct
GGRGYDRLN

SEQ ID NO: 35016 - protein, 9 aa, synthetic construct
GGSGADDIH

SEQ ID NO: 35017 - protein, 9 aa, synthetic construct
GGRGYDTLN

SEQ ID NO: 35018 - protein, 9 aa, synthetic construct
GGRGYDTLT

SEQ ID NO: 35019 - protein, 9 aa, synthetic construct
GGSGADAFD

SEQ ID NO: 35020 - protein, 9 aa, synthetic construct
GGSGADAFT

SEQ ID NO: 35021 - protein, 9 aa, synthetic construct
GGSGADAID

SEQ ID NO: 35022 - protein, 9 aa, synthetic construct
GGSGADALM

SEQ ID NO: 35023 - protein, 9 aa, synthetic construct
GGSGADALN

SEQ ID NO: 35024 - protein, 9 aa, synthetic construct
GGSGADALR

SEQ ID NO: 35025 - protein, 9 aa, synthetic construct
GGSGADAMT

SEQ ID NO: 35026 - protein, 9 aa, synthetic construct
GGSGADAMY

SEQ ID NO: 35027 - protein, 9 aa, synthetic construct
GGSGADCLY

SEQ ID NO: 35028 - protein, 9 aa, synthetic construct
GGSGADDFI

SEQ ID NO: 35029 - protein, 9 aa, synthetic construct
GGSGADDIF

SEQ ID NO: 35030 - protein, 9 aa, synthetic construct
GGRGSDYME

SEQ ID NO: 35031 - protein, 9 aa, synthetic construct
GGRGSDYLL

SEQ ID NO: 35032 - protein, 9 aa, synthetic construct
GGRGSDYLE

SEQ ID NO: 35033 - protein, 9 aa, synthetic construct
GGRGSDYIE

SEQ ID NO: 35034 - protein, 9 aa, synthetic construct
GGRGSDDLD

SEQ ID NO: 35035 - protein, 9 aa, synthetic construct
GGRGSDDLF

SEQ ID NO: 35036 - protein, 9 aa, synthetic construct
GGRGSDEID

SEQ ID NO: 35037 - protein, 9 aa, synthetic construct
GGRGSDELH

SEQ ID NO: 35038 - protein, 9 aa, synthetic construct
GGRGSDELL

SEQ ID NO: 35039 - protein, 9 aa, synthetic construct
GGRGSDELY

SEQ ID NO: 35040 - protein, 9 aa, synthetic construct
GGRGSDEMH

SEQ ID NO: 35041 - protein, 9 aa, synthetic construct
GGRGSDFLA

SEQ ID NO: 35042 - protein, 9 aa, synthetic construct
GGRGSDFLF

SEQ ID NO: 35043 - protein, 9 aa, synthetic construct
GGRGSDFLK

SEQ ID NO: 35044 - protein, 9 aa, synthetic construct
GGRGSDGLF

SEQ ID NO: 35045 - protein, 9 aa, synthetic construct
GGRGSDHFV

SEQ ID NO: 35046 - protein, 9 aa, synthetic construct
GGRGSDHLA

SEQ ID NO: 35047 - protein, 9 aa, synthetic construct
GGRGSDHLD

SEQ ID NO: 35048 - protein, 9 aa, synthetic construct
GGRGSDHLW

SEQ ID NO: 35049 - protein, 9 aa, synthetic construct
GGRGSDILD

SEQ ID NO: 35050 - protein, 9 aa, synthetic construct
GGRGSDILF

SEQ ID NO: 35051 - protein, 9 aa, synthetic construct
GGRGSDILL

SEQ ID NO: 35052 - protein, 9 aa, synthetic construct
GGRGSDILT

SEQ ID NO: 35053 - protein, 9 aa, synthetic construct
GGRGSDILY

SEQ ID NO: 35054 - protein, 9 aa, synthetic construct
GGRGSDIVD

SEQ ID NO: 35055 - protein, 9 aa, synthetic construct
GGRGSDKLD

SEQ ID NO: 35056 - protein, 9 aa, synthetic construct
GGRGSDKMS

SEQ ID NO: 35057 - protein, 9 aa, synthetic construct
GGRGSDLFI

SEQ ID NO: 35058 - protein, 9 aa, synthetic construct
GGRGSDLFM

SEQ ID NO: 35059 - protein, 9 aa, synthetic construct
GGRGSDLIV

SEQ ID NO: 35060 - protein, 9 aa, synthetic construct
GGRGSDLIY

SEQ ID NO: 35061 - protein, 9 aa, synthetic construct
GGRGSDLLF

SEQ ID NO: 35062 - protein, 9 aa, synthetic construct
GGRGSDLLK

SEQ ID NO: 35063 - protein, 9 aa, synthetic construct
GGRGSDALS

SEQ ID NO: 35064 - protein, 9 aa, synthetic construct
GGRGSDALD

SEQ ID NO: 35065 - protein, 9 aa, synthetic construct
GGRGRDYLY

SEQ ID NO: 35066 - protein, 9 aa, synthetic construct
GGRGRDTLS

SEQ ID NO: 35067 - protein, 9 aa, synthetic construct
GGRGRDSIV

SEQ ID NO: 35068 - protein, 9 aa, synthetic construct
GGRGRDSLL

SEQ ID NO: 35069 - protein, 9 aa, synthetic construct
GGRGRDSLQ

SEQ ID NO: 35070 - protein, 9 aa, synthetic construct
GGRGRDSLS

SEQ ID NO: 35071 - protein, 9 aa, synthetic construct
GGRGRDSLY

SEQ ID NO: 35072 - protein, 9 aa, synthetic construct
GGRGRDSMH

SEQ ID NO: 35073 - protein, 9 aa, synthetic construct
GGRGRDTAR

SEQ ID NO: 35074 - protein, 9 aa, synthetic construct
GGRGRDTIA

SEQ ID NO: 35075 - protein, 9 aa, synthetic construct
GGRGRDTII

SEQ ID NO: 35076 - protein, 9 aa, synthetic construct
GGRGRDTIR

SEQ ID NO: 35077 - protein, 9 aa, synthetic construct
GGRGRDTIS

SEQ ID NO: 35078 - protein, 9 aa, synthetic construct
GGRGRDTLD

SEQ ID NO: 35079 - protein, 9 aa, synthetic construct
GGRGRDTLN

SEQ ID NO: 35080 - protein, 9 aa, synthetic construct
GGRGRDTLV

SEQ ID NO: 35081 - protein, 9 aa, synthetic construct
GGRGRDWLS

SEQ ID NO: 35082 - protein, 9 aa, synthetic construct
GGRGRDTVF

SEQ ID NO: 35083 - protein, 9 aa, synthetic construct
GGRGRDVFI

SEQ ID NO: 35084 - protein, 9 aa, synthetic construct
GGRGRDVFT

SEQ ID NO: 35085 - protein, 9 aa, synthetic construct
GGRGRDVID

SEQ ID NO: 35086 - protein, 9 aa, synthetic construct
GGRGRDVIL

SEQ ID NO: 35087 - protein, 9 aa, synthetic construct
GGRGRDVLE

SEQ ID NO: 35088 - protein, 9 aa, synthetic construct
GGRGRDVLK

SEQ ID NO: 35089 - protein, 9 aa, synthetic construct
GGRGRDVLS

SEQ ID NO: 35090 - protein, 9 aa, synthetic construct
GGRGRDVLV

SEQ ID NO: 35091 - protein, 9 aa, synthetic construct
GGRGRDVMQ

SEQ ID NO: 35092 - protein, 9 aa, synthetic construct
GGRGRDVMV

SEQ ID NO: 35093 - protein, 9 aa, synthetic construct
GGRGRDVVL

SEQ ID NO: 35094 - protein, 9 aa, synthetic construct
GGRGRDVYQ

SEQ ID NO: 35095 - protein, 9 aa, synthetic construct
GGRGSDLLL

SEQ ID NO: 35096 - protein, 9 aa, synthetic construct
GGRGSDLLN

SEQ ID NO: 35097 - protein, 9 aa, synthetic construct
GGRGSDLLQ

SEQ ID NO: 35098 - protein, 9 aa, synthetic construct
GGRGSDTMD

SEQ ID NO: 35099 - protein, 9 aa, synthetic construct
GGRGSDSYY

SEQ ID NO: 35100 - protein, 9 aa, synthetic construct
GGRGSDTAS

SEQ ID NO: 35101 - protein, 9 aa, synthetic construct
GGRGSDTFA

SEQ ID NO: 35102 - protein, 9 aa, synthetic construct
GGRGSDTFH

SEQ ID NO: 35103 - protein, 9 aa, synthetic construct
GGRGSDTFL

SEQ ID NO: 35104 - protein, 9 aa, synthetic construct
GGRGSDTFY

SEQ ID NO: 35105 - protein, 9 aa, synthetic construct
GGRGSDTIF

SEQ ID NO: 35106 - protein, 9 aa, synthetic construct
GGRGSDTII

SEQ ID NO: 35107 - protein, 9 aa, synthetic construct
GGRGSDTIN

SEQ ID NO: 35108 - protein, 9 aa, synthetic construct
GGRGSDTIS

SEQ ID NO: 35109 - protein, 9 aa, synthetic construct
GGRGSDTIY

SEQ ID NO: 35110 - protein, 9 aa, synthetic construct
GGRGSDTLE

SEQ ID NO: 35111 - protein, 9 aa, synthetic construct
GGRGSDTLN

SEQ ID NO: 35112 - protein, 9 aa, synthetic construct
GGRGSDTML

SEQ ID NO: 35113 - protein, 9 aa, synthetic construct
GGRGSDSLS

SEQ ID NO: 35114 - protein, 9 aa, synthetic construct
GGRGSDTVS

SEQ ID NO: 35115 - protein, 9 aa, synthetic construct
GGRGSDTYS

SEQ ID NO: 35116 - protein, 9 aa, synthetic construct
GGRGSDVFA

SEQ ID NO: 35117 - protein, 9 aa, synthetic construct
GGRGSDVLF

SEQ ID NO: 35118 - protein, 9 aa, synthetic construct
GGRGSDVLH

SEQ ID NO: 35119 - protein, 9 aa, synthetic construct
GGRGSDVLN

SEQ ID NO: 35120 - protein, 9 aa, synthetic construct
GGRGSDVLQ

SEQ ID NO: 35121 - protein, 9 aa, synthetic construct
GGRGSDVLR

SEQ ID NO: 35122 - protein, 9 aa, synthetic construct
GGRGSDVLV

SEQ ID NO: 35123 - protein, 9 aa, synthetic construct
GGRGSDVMV

SEQ ID NO: 35124 - protein, 9 aa, synthetic construct
GGRGSDWII

SEQ ID NO: 35125 - protein, 9 aa, synthetic construct
GGRGSDWLM

SEQ ID NO: 35126 - protein, 9 aa, synthetic construct
GGRGSDWMD

SEQ ID NO: 35127 - protein, 9 aa, synthetic construct
GGRGSDSYF

SEQ ID NO: 35128 - protein, 9 aa, synthetic construct
GGRGSDSLM

SEQ ID NO: 35129 - protein, 9 aa, synthetic construct
GGRGSDLLV

SEQ ID NO: 35130 - protein, 9 aa, synthetic construct
GGRGSDRIL

SEQ ID NO: 35131 - protein, 9 aa, synthetic construct
GGRGSDLLY

SEQ ID NO: 35132 - protein, 9 aa, synthetic construct
GGRGSDLMT

SEQ ID NO: 35133 - protein, 9 aa, synthetic construct
GGRGSDMID

SEQ ID NO: 35134 - protein, 9 aa, synthetic construct
GGRGSDMLD

SEQ ID NO: 35135 - protein, 9 aa, synthetic construct
GGRGSDMLL

SEQ ID NO: 35136 - protein, 9 aa, synthetic construct
GGRGSDMLV

SEQ ID NO: 35137 - protein, 9 aa, synthetic construct
GGRGSDNLF

SEQ ID NO: 35138 - protein, 9 aa, synthetic construct
GGRGSDQIL

SEQ ID NO: 35139 - protein, 9 aa, synthetic construct
GGRGSDQLN

SEQ ID NO: 35140 - protein, 9 aa, synthetic construct
GGRGSDQLS

SEQ ID NO: 35141 - protein, 9 aa, synthetic construct
GGRGSDQLY

SEQ ID NO: 35142 - protein, 9 aa, synthetic construct
GGRGSDRFV

SEQ ID NO: 35143 - protein, 9 aa, synthetic construct
GGRGSDRIE

SEQ ID NO: 35144 - protein, 9 aa, synthetic construct
GGRGSDRIR

SEQ ID NO: 35145 - protein, 9 aa, synthetic construct
GGRGSDSLD

SEQ ID NO: 35146 - protein, 9 aa, synthetic construct
GGRGSDRLA

SEQ ID NO: 35147 - protein, 9 aa, synthetic construct
GGRGSDRLE

SEQ ID NO: 35148 - protein, 9 aa, synthetic construct
GGRGSDRLR

SEQ ID NO: 35149 - protein, 9 aa, synthetic construct
GGRGSDRLS

SEQ ID NO: 35150 - protein, 9 aa, synthetic construct
GGRGSDRLT

SEQ ID NO: 35151 - protein, 9 aa, synthetic construct
GGRGSDRLW

SEQ ID NO: 35152 - protein, 9 aa, synthetic construct
GGRGSDRLY

SEQ ID NO: 35153 - protein, 9 aa, synthetic construct
GGRGSDRYI

SEQ ID NO: 35154 - protein, 9 aa, synthetic construct
GGRGSDRYL

SEQ ID NO: 35155 - protein, 9 aa, synthetic construct
GGRGSDSIL

SEQ ID NO: 35156 - protein, 9 aa, synthetic construct
GGRGSDSIN

SEQ ID NO: 35157 - protein, 9 aa, synthetic construct
GGRGSDSIS

SEQ ID NO: 35158 - protein, 9 aa, synthetic construct
GGRGSDSLA

SEQ ID NO: 35159 - protein, 9 aa, synthetic construct
GGSGEDIFR

SEQ ID NO: 35160 - protein, 9 aa, synthetic construct
GGSGEDIIR

SEQ ID NO: 35161 - protein, 9 aa, synthetic construct
GGSGEDIIS

SEQ ID NO: 35162 - protein, 9 aa, synthetic construct
GGSGNDKME

SEQ ID NO: 35163 - protein, 9 aa, synthetic construct
GGSGNDHLG

SEQ ID NO: 35164 - protein, 9 aa, synthetic construct
GGSGNDHLK

SEQ ID NO: 35165 - protein, 9 aa, synthetic construct
GGSGNDHLV

SEQ ID NO: 35166 - protein, 9 aa, synthetic construct
GGSGNDHVQ

SEQ ID NO: 35167 - protein, 9 aa, synthetic construct
GGSGNDIAI

SEQ ID NO: 35168 - protein, 9 aa, synthetic construct
GGSGNDIAK

SEQ ID NO: 35169 - protein, 9 aa, synthetic construct
GGSGNDIFD

SEQ ID NO: 35170 - protein, 9 aa, synthetic construct
GGSGNDIFE

SEQ ID NO: 35171 - protein, 9 aa, synthetic construct
GGSGNDIFF

SEQ ID NO: 35172 - protein, 9 aa, synthetic construct
GGSGNDIFR

SEQ ID NO: 35173 - protein, 9 aa, synthetic construct
GGSGNDIFT

SEQ ID NO: 35174 - protein, 9 aa, synthetic construct
GGSGNDIIG

SEQ ID NO: 35175 - protein, 9 aa, synthetic construct
GGSGNDIIM

SEQ ID NO: 35176 - protein, 9 aa, synthetic construct
GGSGNDIIN

SEQ ID NO: 35177 - protein, 9 aa, synthetic construct
GGSGNDIIR

SEQ ID NO: 35178 - protein, 9 aa, synthetic construct
GGSGNDILM

SEQ ID NO: 35179 - protein, 9 aa, synthetic construct
GGSGNDIMD

SEQ ID NO: 35180 - protein, 9 aa, synthetic construct
GGSGNDIME

SEQ ID NO: 35181 - protein, 9 aa, synthetic construct
GGSGNDIMR

SEQ ID NO: 35182 - protein, 9 aa, synthetic construct
GGSGNDIMS

SEQ ID NO: 35183 - protein, 9 aa, synthetic construct
GGSGNDIMT

SEQ ID NO: 35184 - protein, 9 aa, synthetic construct
GGSGNDIMY

SEQ ID NO: 35185 - protein, 9 aa, synthetic construct
GGSGNDIVA

SEQ ID NO: 35186 - protein, 9 aa, synthetic construct
GGSGNDIVI

SEQ ID NO: 35187 - protein, 9 aa, synthetic construct
GGSGNDIVL

SEQ ID NO: 35188 - protein, 9 aa, synthetic construct
GGSGNDKAT

SEQ ID NO: 35189 - protein, 9 aa, synthetic construct
GGSGNDKFN

SEQ ID NO: 35190 - protein, 9 aa, synthetic construct
GGSGNDKIK

SEQ ID NO: 35191 - protein, 9 aa, synthetic construct
GGSGNDKIL

SEQ ID NO: 35192 - protein, 9 aa, synthetic construct
GGSGNDHIN

SEQ ID NO: 35193 - protein, 9 aa, synthetic construct
GGSGNDHIL

SEQ ID NO: 35194 - protein, 9 aa, synthetic construct
GGSGNDHII

SEQ ID NO: 35195 - protein, 9 aa, synthetic construct
GGSGNDFVC

SEQ ID NO: 35196 - protein, 9 aa, synthetic construct
GGSGNDFFI

SEQ ID NO: 35197 - protein, 9 aa, synthetic construct
GGSGNDFFV

SEQ ID NO: 35198 - protein, 9 aa, synthetic construct
GGSGNDFIA

SEQ ID NO: 35199 - protein, 9 aa, synthetic construct
GGSGNDFIF

SEQ ID NO: 35200 - protein, 9 aa, synthetic construct
GGSGNDFIK

SEQ ID NO: 35201 - protein, 9 aa, synthetic construct
GGSGNDFIT

SEQ ID NO: 35202 - protein, 9 aa, synthetic construct
GGSGNDFIY

SEQ ID NO: 35203 - protein, 9 aa, synthetic construct
GGSGNDFLG

SEQ ID NO: 35204 - protein, 9 aa, synthetic construct
GGSGNDFLK

SEQ ID NO: 35205 - protein, 9 aa, synthetic construct
GGSGNDFMD

SEQ ID NO: 35206 - protein, 9 aa, synthetic construct
GGSGNDFMR

SEQ ID NO: 35207 - protein, 9 aa, synthetic construct
GGSGNDFMT

SEQ ID NO: 35208 - protein, 9 aa, synthetic construct
GGSGNDFMY

SEQ ID NO: 35209 - protein, 9 aa, synthetic construct
GGSGNDFVD

SEQ ID NO: 35210 - protein, 9 aa, synthetic construct
GGSGNDHFY

SEQ ID NO: 35211 - protein, 9 aa, synthetic construct
GGSGNDFVN

SEQ ID NO: 35212 - protein, 9 aa, synthetic construct
GGSGNDFVQ

SEQ ID NO: 35213 - protein, 9 aa, synthetic construct
GGSGNDFYT

SEQ ID NO: 35214 - protein, 9 aa, synthetic construct
GGSGNDFYV

SEQ ID NO: 35215 - protein, 9 aa, synthetic construct
GGSGNDGFG

SEQ ID NO: 35216 - protein, 9 aa, synthetic construct
GGSGNDGID

SEQ ID NO: 35217 - protein, 9 aa, synthetic construct
GGSGNDGLA

SEQ ID NO: 35218 - protein, 9 aa, synthetic construct
GGSGNDGLN

SEQ ID NO: 35219 - protein, 9 aa, synthetic construct
GGSGNDGLS

SEQ ID NO: 35220 - protein, 9 aa, synthetic construct
GGSGNDGVA

SEQ ID NO: 35221 - protein, 9 aa, synthetic construct
GGSGNDHAT

SEQ ID NO: 35222 - protein, 9 aa, synthetic construct
GGSGNDHAY

SEQ ID NO: 35223 - protein, 9 aa, synthetic construct
GGSGNDHFI

SEQ ID NO: 35224 - protein, 9 aa, synthetic construct
GGSGNDKIS

SEQ ID NO: 35225 - protein, 9 aa, synthetic construct
GGSGNDKMI

SEQ ID NO: 35226 - protein, 9 aa, synthetic construct
GGSGNDRFQ

SEQ ID NO: 35227 - protein, 9 aa, synthetic construct
GGSGNDKVE

SEQ ID NO: 35228 - protein, 9 aa, synthetic construct
GGSGNDNIK

SEQ ID NO: 35229 - protein, 9 aa, synthetic construct
GGSGNDNIL

SEQ ID NO: 35230 - protein, 9 aa, synthetic construct
GGSGNDNIN

SEQ ID NO: 35231 - protein, 9 aa, synthetic construct
GGSGNDNLE

SEQ ID NO: 35232 - protein, 9 aa, synthetic construct
GGSGNDNLH

SEQ ID NO: 35233 - protein, 9 aa, synthetic construct
GGSGNDNLV

SEQ ID NO: 35234 - protein, 9 aa, synthetic construct
GGSGNDNMH

SEQ ID NO: 35235 - protein, 9 aa, synthetic construct
GGSGNDNVD

SEQ ID NO: 35236 - protein, 9 aa, synthetic construct
GGSGNDNVF

SEQ ID NO: 35237 - protein, 9 aa, synthetic construct
GGSGNDNYL

SEQ ID NO: 35238 - protein, 9 aa, synthetic construct
GGSGNDQFA

SEQ ID NO: 35239 - protein, 9 aa, synthetic construct
GGSGNDQFF

SEQ ID NO: 35240 - protein, 9 aa, synthetic construct
GGSGNDQFI

SEQ ID NO: 35241 - protein, 9 aa, synthetic construct
GGSGNDQID

SEQ ID NO: 35242 - protein, 9 aa, synthetic construct
GGSGNDQIE

SEQ ID NO: 35243 - protein, 9 aa, synthetic construct
GGSGNDQIK

SEQ ID NO: 35244 - protein, 9 aa, synthetic construct
GGSGNDQIM

SEQ ID NO: 35245 - protein, 9 aa, synthetic construct
GGSGNDQIN

SEQ ID NO: 35246 - protein, 9 aa, synthetic construct
GGSGNDQIQ

SEQ ID NO: 35247 - protein, 9 aa, synthetic construct
GGSGNDQIR

SEQ ID NO: 35248 - protein, 9 aa, synthetic construct
GGSGNDQIT

SEQ ID NO: 35249 - protein, 9 aa, synthetic construct
GGSGNDQMH

SEQ ID NO: 35250 - protein, 9 aa, synthetic construct
GGSGNDQMN

SEQ ID NO: 35251 - protein, 9 aa, synthetic construct
GGSGNDQMW

SEQ ID NO: 35252 - protein, 9 aa, synthetic construct
GGSGNDQMY

SEQ ID NO: 35253 - protein, 9 aa, synthetic construct
GGSGNDQVN

SEQ ID NO: 35254 - protein, 9 aa, synthetic construct
GGSGNDQVY

SEQ ID NO: 35255 - protein, 9 aa, synthetic construct
GGSGNDRAS

SEQ ID NO: 35256 - protein, 9 aa, synthetic construct
GGSGNDRAY

SEQ ID NO: 35257 - protein, 9 aa, synthetic construct
GGSGNDNIH

SEQ ID NO: 35258 - protein, 9 aa, synthetic construct
GGSGNDNIE

SEQ ID NO: 35259 - protein, 9 aa, synthetic construct
GGSGNDNAF

SEQ ID NO: 35260 - protein, 9 aa, synthetic construct
GGSGNDLYK

SEQ ID NO: 35261 - protein, 9 aa, synthetic construct
GGSGNDKVF

SEQ ID NO: 35262 - protein, 9 aa, synthetic construct
GGSGNDLFT

SEQ ID NO: 35263 - protein, 9 aa, synthetic construct
GGSGNDLIH

SEQ ID NO: 35264 - protein, 9 aa, synthetic construct
GGSGNDLIK

SEQ ID NO: 35265 - protein, 9 aa, synthetic construct
GGSGNDLLG

SEQ ID NO: 35266 - protein, 9 aa, synthetic construct
GGSGNDLMI

SEQ ID NO: 35267 - protein, 9 aa, synthetic construct
GGSGNDLML

SEQ ID NO: 35268 - protein, 9 aa, synthetic construct
GGSGNDLMQ

SEQ ID NO: 35269 - protein, 9 aa, synthetic construct
GGSGNDLMW

SEQ ID NO: 35270 - protein, 9 aa, synthetic construct
GGSGNDLVH

SEQ ID NO: 35271 - protein, 9 aa, synthetic construct
GGSGNDLVM

SEQ ID NO: 35272 - protein, 9 aa, synthetic construct
GGSGNDLVV

SEQ ID NO: 35273 - protein, 9 aa, synthetic construct
GGSGNDLVW

SEQ ID NO: 35274 - protein, 9 aa, synthetic construct
GGSGNDLYN

SEQ ID NO: 35275 - protein, 9 aa, synthetic construct
GGSGNDMVV

SEQ ID NO: 35276 - protein, 9 aa, synthetic construct
GGSGNDMFD

SEQ ID NO: 35277 - protein, 9 aa, synthetic construct
GGSGNDMFI

SEQ ID NO: 35278 - protein, 9 aa, synthetic construct
GGSGNDMFR

SEQ ID NO: 35279 - protein, 9 aa, synthetic construct
GGSGNDMFY

SEQ ID NO: 35280 - protein, 9 aa, synthetic construct
GGSGNDMIF

SEQ ID NO: 35281 - protein, 9 aa, synthetic construct
GGSGNDMIT

SEQ ID NO: 35282 - protein, 9 aa, synthetic construct
GGSGNDMIV

SEQ ID NO: 35283 - protein, 9 aa, synthetic construct
GGSGNDMLE

SEQ ID NO: 35284 - protein, 9 aa, synthetic construct
GGSGNDMLI

SEQ ID NO: 35285 - protein, 9 aa, synthetic construct
GGSGNDMLK

SEQ ID NO: 35286 - protein, 9 aa, synthetic construct
GGSGNDMMF

SEQ ID NO: 35287 - protein, 9 aa, synthetic construct
GGSGNDMMV

SEQ ID NO: 35288 - protein, 9 aa, synthetic construct
GGSGNDMVF

SEQ ID NO: 35289 - protein, 9 aa, synthetic construct
GGSGNDFFF

SEQ ID NO: 35290 - protein, 9 aa, synthetic construct
GGSGNDFAI

SEQ ID NO: 35291 - protein, 9 aa, synthetic construct
GGSGNDEYR

SEQ ID NO: 35292 - protein, 9 aa, synthetic construct
GGSGNDEVT

SEQ ID NO: 35293 - protein, 9 aa, synthetic construct
GGSGLDVFV

SEQ ID NO: 35294 - protein, 9 aa, synthetic construct
GGSGLDVIF

SEQ ID NO: 35295 - protein, 9 aa, synthetic construct
GGSGLDVLF

SEQ ID NO: 35296 - protein, 9 aa, synthetic construct
GGSGLDVLT

SEQ ID NO: 35297 - protein, 9 aa, synthetic construct
GGSGLDVLV

SEQ ID NO: 35298 - protein, 9 aa, synthetic construct
GGSGLDVMF

SEQ ID NO: 35299 - protein, 9 aa, synthetic construct
GGSGLDVMM

SEQ ID NO: 35300 - protein, 9 aa, synthetic construct
GGSGLDVYE

SEQ ID NO: 35301 - protein, 9 aa, synthetic construct
GGSGLDVYT

SEQ ID NO: 35302 - protein, 9 aa, synthetic construct
GGSGLDWAL

SEQ ID NO: 35303 - protein, 9 aa, synthetic construct
GGSGLDWFY

SEQ ID NO: 35304 - protein, 9 aa, synthetic construct
GGSGLDWLL

SEQ ID NO: 35305 - protein, 9 aa, synthetic construct
GGSGLDYLN

SEQ ID NO: 35306 - protein, 9 aa, synthetic construct
GGSGLDYLV

SEQ ID NO: 35307 - protein, 9 aa, synthetic construct
GGSGMDFFD

SEQ ID NO: 35308 - protein, 9 aa, synthetic construct
GGSGMDFLD

SEQ ID NO: 35309 - protein, 9 aa, synthetic construct
GGSGMDFVD

SEQ ID NO: 35310 - protein, 9 aa, synthetic construct
GGSGMDHLA

SEQ ID NO: 35311 - protein, 9 aa, synthetic construct
GGSGMDHLE

SEQ ID NO: 35312 - protein, 9 aa, synthetic construct
GGSGMDIIS

SEQ ID NO: 35313 - protein, 9 aa, synthetic construct
GGSGMDILN

SEQ ID NO: 35314 - protein, 9 aa, synthetic construct
GGSGMDKLF

SEQ ID NO: 35315 - protein, 9 aa, synthetic construct
GGSGMDKLI

SEQ ID NO: 35316 - protein, 9 aa, synthetic construct
GGSGMDMMK

SEQ ID NO: 35317 - protein, 9 aa, synthetic construct
GGSGMDQID

SEQ ID NO: 35318 - protein, 9 aa, synthetic construct
GGSGMDRLY

SEQ ID NO: 35319 - protein, 9 aa, synthetic construct
GGSGMDRMF

SEQ ID NO: 35320 - protein, 9 aa, synthetic construct
GGSGMDTAV

SEQ ID NO: 35321 - protein, 9 aa, synthetic construct
GGSGMDTFV

SEQ ID NO: 35322 - protein, 9 aa, synthetic construct
GGSGLDVFT

SEQ ID NO: 35323 - protein, 9 aa, synthetic construct
GGSGLDVAQ

SEQ ID NO: 35324 - protein, 9 aa, synthetic construct
GGSGLDVAL

SEQ ID NO: 35325 - protein, 9 aa, synthetic construct
GGSGLDRFI

SEQ ID NO: 35326 - protein, 9 aa, synthetic construct
GGSGLDKLT

SEQ ID NO: 35327 - protein, 9 aa, synthetic construct
GGSGLDKLY

SEQ ID NO: 35328 - protein, 9 aa, synthetic construct
GGSGLDLIY

SEQ ID NO: 35329 - protein, 9 aa, synthetic construct
GGSGLDLLI

SEQ ID NO: 35330 - protein, 9 aa, synthetic construct
GGSGLDLLV

SEQ ID NO: 35331 - protein, 9 aa, synthetic construct
GGSGLDNLA

SEQ ID NO: 35332 - protein, 9 aa, synthetic construct
GGSGLDNLQ

SEQ ID NO: 35333 - protein, 9 aa, synthetic construct
GGSGLDQFV

SEQ ID NO: 35334 - protein, 9 aa, synthetic construct
GGSGLDQLD

SEQ ID NO: 35335 - protein, 9 aa, synthetic construct
GGSGLDQLI

SEQ ID NO: 35336 - protein, 9 aa, synthetic construct
GGSGLDQLY

SEQ ID NO: 35337 - protein, 9 aa, synthetic construct
GGSGLDQVL

SEQ ID NO: 35338 - protein, 9 aa, synthetic construct
GGSGLDRAH

SEQ ID NO: 35339 - protein, 9 aa, synthetic construct
GGSGLDRLK

SEQ ID NO: 35340 - protein, 9 aa, synthetic construct
GGSGLDVAI

SEQ ID NO: 35341 - protein, 9 aa, synthetic construct
GGSGLDSLD

SEQ ID NO: 35342 - protein, 9 aa, synthetic construct
GGSGLDSLT

SEQ ID NO: 35343 - protein, 9 aa, synthetic construct
GGSGLDSLV

SEQ ID NO: 35344 - protein, 9 aa, synthetic construct
GGSGLDTAS

SEQ ID NO: 35345 - protein, 9 aa, synthetic construct
GGSGLDTAV

SEQ ID NO: 35346 - protein, 9 aa, synthetic construct
GGSGLDTFI

SEQ ID NO: 35347 - protein, 9 aa, synthetic construct
GGSGLDTID

SEQ ID NO: 35348 - protein, 9 aa, synthetic construct
GGSGLDTIT

SEQ ID NO: 35349 - protein, 9 aa, synthetic construct
GGSGLDTLH

SEQ ID NO: 35350 - protein, 9 aa, synthetic construct
GGSGLDTLI

SEQ ID NO: 35351 - protein, 9 aa, synthetic construct
GGSGLDTLS

SEQ ID NO: 35352 - protein, 9 aa, synthetic construct
GGSGLDTLW

SEQ ID NO: 35353 - protein, 9 aa, synthetic construct
GGSGLDTMN

SEQ ID NO: 35354 - protein, 9 aa, synthetic construct
GGSGMDTLW

SEQ ID NO: 35355 - protein, 9 aa, synthetic construct
GGSGMDTMS

SEQ ID NO: 35356 - protein, 9 aa, synthetic construct
GGSGMDVLA

SEQ ID NO: 35357 - protein, 9 aa, synthetic construct
GGSGNDDYI

SEQ ID NO: 35358 - protein, 9 aa, synthetic construct
GGSGNDDFI

SEQ ID NO: 35359 - protein, 9 aa, synthetic construct
GGSGNDDIA

SEQ ID NO: 35360 - protein, 9 aa, synthetic construct
GGSGNDDIF

SEQ ID NO: 35361 - protein, 9 aa, synthetic construct
GGSGNDDLA

SEQ ID NO: 35362 - protein, 9 aa, synthetic construct
GGSGNDDLK

SEQ ID NO: 35363 - protein, 9 aa, synthetic construct
GGSGNDDLW

SEQ ID NO: 35364 - protein, 9 aa, synthetic construct
GGSGNDDMD

SEQ ID NO: 35365 - protein, 9 aa, synthetic construct
GGSGNDDMG

SEQ ID NO: 35366 - protein, 9 aa, synthetic construct
GGSGNDDVD

SEQ ID NO: 35367 - protein, 9 aa, synthetic construct
GGSGNDDVH

SEQ ID NO: 35368 - protein, 9 aa, synthetic construct
GGSGNDDVN

SEQ ID NO: 35369 - protein, 9 aa, synthetic construct
GGSGNDDVR

SEQ ID NO: 35370 - protein, 9 aa, synthetic construct
GGSGNDDYH

SEQ ID NO: 35371 - protein, 9 aa, synthetic construct
GGSGNDEFA

SEQ ID NO: 35372 - protein, 9 aa, synthetic construct
GGSGNDCLE

SEQ ID NO: 35373 - protein, 9 aa, synthetic construct
GGSGNDEFR

SEQ ID NO: 35374 - protein, 9 aa, synthetic construct
GGSGNDEID

SEQ ID NO: 35375 - protein, 9 aa, synthetic construct
GGSGNDEIN

SEQ ID NO: 35376 - protein, 9 aa, synthetic construct
GGSGNDELH

SEQ ID NO: 35377 - protein, 9 aa, synthetic construct
GGSGNDEMH

SEQ ID NO: 35378 - protein, 9 aa, synthetic construct
GGSGNDEMK

SEQ ID NO: 35379 - protein, 9 aa, synthetic construct
GGSGNDEMR

SEQ ID NO: 35380 - protein, 9 aa, synthetic construct
GGSGNDEMT

SEQ ID NO: 35381 - protein, 9 aa, synthetic construct
GGSGNDEMW

SEQ ID NO: 35382 - protein, 9 aa, synthetic construct
GGSGNDEMY

SEQ ID NO: 35383 - protein, 9 aa, synthetic construct
GGSGNDEVF

SEQ ID NO: 35384 - protein, 9 aa, synthetic construct
GGSGNDEVI

SEQ ID NO: 35385 - protein, 9 aa, synthetic construct
GGSGNDEVM

SEQ ID NO: 35386 - protein, 9 aa, synthetic construct
GGSGNDCLL

SEQ ID NO: 35387 - protein, 9 aa, synthetic construct
GGSGNDCLA

SEQ ID NO: 35388 - protein, 9 aa, synthetic construct
GGSGMDVMY

SEQ ID NO: 35389 - protein, 9 aa, synthetic construct
GGSGNDALG

SEQ ID NO: 35390 - protein, 9 aa, synthetic construct
GGSGMDWIE

SEQ ID NO: 35391 - protein, 9 aa, synthetic construct
GGSGMDYAS

SEQ ID NO: 35392 - protein, 9 aa, synthetic construct
GGSGMDYLD

SEQ ID NO: 35393 - protein, 9 aa, synthetic construct
GGSGMDYLS

SEQ ID NO: 35394 - protein, 9 aa, synthetic construct
GGSGMDYMA

SEQ ID NO: 35395 - protein, 9 aa, synthetic construct
GGSGNDAFA

SEQ ID NO: 35396 - protein, 9 aa, synthetic construct
GGSGNDAFF

SEQ ID NO: 35397 - protein, 9 aa, synthetic construct
GGSGNDAFV

SEQ ID NO: 35398 - protein, 9 aa, synthetic construct
GGSGNDAIA

SEQ ID NO: 35399 - protein, 9 aa, synthetic construct
GGSGNDAIK

SEQ ID NO: 35400 - protein, 9 aa, synthetic construct
GGSGNDAIR

SEQ ID NO: 35401 - protein, 9 aa, synthetic construct
GGSGNDAIV

SEQ ID NO: 35402 - protein, 9 aa, synthetic construct
GGSGNDAIY

SEQ ID NO: 35403 - protein, 9 aa, synthetic construct
GGSGNDALV

SEQ ID NO: 35404 - protein, 9 aa, synthetic construct
GGSGNDCIS

SEQ ID NO: 35405 - protein, 9 aa, synthetic construct
GGSGNDAMH

SEQ ID NO: 35406 - protein, 9 aa, synthetic construct
GGSGNDAMI

SEQ ID NO: 35407 - protein, 9 aa, synthetic construct
GGSGNDAMR

SEQ ID NO: 35408 - protein, 9 aa, synthetic construct
GGSGNDAMY

SEQ ID NO: 35409 - protein, 9 aa, synthetic construct
GGSGNDAVL

SEQ ID NO: 35410 - protein, 9 aa, synthetic construct
GGSGNDAVN

SEQ ID NO: 35411 - protein, 9 aa, synthetic construct
GGSGNDAVQ

SEQ ID NO: 35412 - protein, 9 aa, synthetic construct
GGSGNDAVS

SEQ ID NO: 35413 - protein, 9 aa, synthetic construct
GGSGNDAVY

SEQ ID NO: 35414 - protein, 9 aa, synthetic construct
GGSGNDAYD

SEQ ID NO: 35415 - protein, 9 aa, synthetic construct
GGSGNDAYI

SEQ ID NO: 35416 - protein, 9 aa, synthetic construct
GGSGNDAYT

SEQ ID NO: 35417 - protein, 9 aa, synthetic construct
GGSGNDCID

SEQ ID NO: 35418 - protein, 9 aa, synthetic construct
GGSGNDRFH

SEQ ID NO: 35419 - protein, 9 aa, synthetic construct
GGSGNDRFR

SEQ ID NO: 35420 - protein, 9 aa, synthetic construct
GGSGEDILR

SEQ ID NO: 35421 - protein, 9 aa, synthetic construct
GGSGQDTYY

SEQ ID NO: 35422 - protein, 9 aa, synthetic construct
GGSGQDQAI

SEQ ID NO: 35423 - protein, 9 aa, synthetic construct
GGSGQDQIR

SEQ ID NO: 35424 - protein, 9 aa, synthetic construct
GGSGQDQLI

SEQ ID NO: 35425 - protein, 9 aa, synthetic construct
GGSGQDQLL

SEQ ID NO: 35426 - protein, 9 aa, synthetic construct
GGSGQDQMD

SEQ ID NO: 35427 - protein, 9 aa, synthetic construct
GGSGQDQVL

SEQ ID NO: 35428 - protein, 9 aa, synthetic construct
GGSGQDRFA

SEQ ID NO: 35429 - protein, 9 aa, synthetic construct
GGSGQDRLD

SEQ ID NO: 35430 - protein, 9 aa, synthetic construct
GGSGQDRLF

SEQ ID NO: 35431 - protein, 9 aa, synthetic construct
GGSGQDRLH

SEQ ID NO: 35432 - protein, 9 aa, synthetic construct
GGSGQDRLL

SEQ ID NO: 35433 - protein, 9 aa, synthetic construct
GGSGQDRLV

SEQ ID NO: 35434 - protein, 9 aa, synthetic construct
GGSGQDSFY

SEQ ID NO: 35435 - protein, 9 aa, synthetic construct
GGSGQDSID

SEQ ID NO: 35436 - protein, 9 aa, synthetic construct
GGSGQDSIF

SEQ ID NO: 35437 - protein, 9 aa, synthetic construct
GGSGQDSIY

SEQ ID NO: 35438 - protein, 9 aa, synthetic construct
GGSGQDSLY

SEQ ID NO: 35439 - protein, 9 aa, synthetic construct
GGSGQDTAD

SEQ ID NO: 35440 - protein, 9 aa, synthetic construct
GGSGQDTAR

SEQ ID NO: 35441 - protein, 9 aa, synthetic construct
GGSGQDTAV

SEQ ID NO: 35442 - protein, 9 aa, synthetic construct
GGSGQDTFK

SEQ ID NO: 35443 - protein, 9 aa, synthetic construct
GGSGQDTIE

SEQ ID NO: 35444 - protein, 9 aa, synthetic construct
GGSGQDTIL

SEQ ID NO: 35445 - protein, 9 aa, synthetic construct
GGSGQDTIW

SEQ ID NO: 35446 - protein, 9 aa, synthetic construct
GGSGQDTLH

SEQ ID NO: 35447 - protein, 9 aa, synthetic construct
GGSGQDTLL

SEQ ID NO: 35448 - protein, 9 aa, synthetic construct
GGSGQDTLR

SEQ ID NO: 35449 - protein, 9 aa, synthetic construct
GGSGQDTVE

SEQ ID NO: 35450 - protein, 9 aa, synthetic construct
GGSGQDTVL

SEQ ID NO: 35451 - protein, 9 aa, synthetic construct
GGSGQDNLS

SEQ ID NO: 35452 - protein, 9 aa, synthetic construct
GGSGQDNLR

SEQ ID NO: 35453 - protein, 9 aa, synthetic construct
GGSGQDNLH

SEQ ID NO: 35454 - protein, 9 aa, synthetic construct
GGSGQDIAD

SEQ ID NO: 35455 - protein, 9 aa, synthetic construct
GGSGQDAFR

SEQ ID NO: 35456 - protein, 9 aa, synthetic construct
GGSGQDAFV

SEQ ID NO: 35457 - protein, 9 aa, synthetic construct
GGSGQDDLR

SEQ ID NO: 35458 - protein, 9 aa, synthetic construct
GGSGQDDVR

SEQ ID NO: 35459 - protein, 9 aa, synthetic construct
GGSGQDDVV

SEQ ID NO: 35460 - protein, 9 aa, synthetic construct
GGSGQDELF

SEQ ID NO: 35461 - protein, 9 aa, synthetic construct
GGSGQDELQ

SEQ ID NO: 35462 - protein, 9 aa, synthetic construct
GGSGQDEMH

SEQ ID NO: 35463 - protein, 9 aa, synthetic construct
GGSGQDFLS

SEQ ID NO: 35464 - protein, 9 aa, synthetic construct
GGSGQDFVK

SEQ ID NO: 35465 - protein, 9 aa, synthetic construct
GGSGQDFVV

SEQ ID NO: 35466 - protein, 9 aa, synthetic construct
GGSGQDHLA

SEQ ID NO: 35467 - protein, 9 aa, synthetic construct
GGSGQDHVH

SEQ ID NO: 35468 - protein, 9 aa, synthetic construct
GGSGQDIAL

SEQ ID NO: 35469 - protein, 9 aa, synthetic construct
GGSGQDNLD

SEQ ID NO: 35470 - protein, 9 aa, synthetic construct
GGSGQDIFV

SEQ ID NO: 35471 - protein, 9 aa, synthetic construct
GGSGQDILK

SEQ ID NO: 35472 - protein, 9 aa, synthetic construct
GGSGQDILW

SEQ ID NO: 35473 - protein, 9 aa, synthetic construct
GGSGQDKIF

SEQ ID NO: 35474 - protein, 9 aa, synthetic construct
GGSGQDKIY

SEQ ID NO: 35475 - protein, 9 aa, synthetic construct
GGSGQDKLY

SEQ ID NO: 35476 - protein, 9 aa, synthetic construct
GGSGQDLFY

SEQ ID NO: 35477 - protein, 9 aa, synthetic construct
GGSGQDLIY

SEQ ID NO: 35478 - protein, 9 aa, synthetic construct
GGSGQDLLD

SEQ ID NO: 35479 - protein, 9 aa, synthetic construct
GGSGQDLLE

SEQ ID NO: 35480 - protein, 9 aa, synthetic construct
GGSGQDMLT

SEQ ID NO: 35481 - protein, 9 aa, synthetic construct
GGSGQDMLY

SEQ ID NO: 35482 - protein, 9 aa, synthetic construct
GGSGQDNID

SEQ ID NO: 35483 - protein, 9 aa, synthetic construct
GGSGQDTYF

SEQ ID NO: 35484 - protein, 9 aa, synthetic construct
GGSGQDVAD

SEQ ID NO: 35485 - protein, 9 aa, synthetic construct
GGSGNDRFT

SEQ ID NO: 35486 - protein, 9 aa, synthetic construct
GGSGQDVFL

SEQ ID NO: 35487 - protein, 9 aa, synthetic construct
GGSGRDFAE

SEQ ID NO: 35488 - protein, 9 aa, synthetic construct
GGSGRDFAR

SEQ ID NO: 35489 - protein, 9 aa, synthetic construct
GGSGRDFLL

SEQ ID NO: 35490 - protein, 9 aa, synthetic construct
GGSGRDFLR

SEQ ID NO: 35491 - protein, 9 aa, synthetic construct
GGSGRDFLS

SEQ ID NO: 35492 - protein, 9 aa, synthetic construct
GGSGRDFLV

SEQ ID NO: 35493 - protein, 9 aa, synthetic construct
GGSGRDFMD

SEQ ID NO: 35494 - protein, 9 aa, synthetic construct
GGSGRDFMY

SEQ ID NO: 35495 - protein, 9 aa, synthetic construct
GGSGRDFVK

SEQ ID NO: 35496 - protein, 9 aa, synthetic construct
GGSGRDFVS

SEQ ID NO: 35497 - protein, 9 aa, synthetic construct
GGSGRDHFM

SEQ ID NO: 35498 - protein, 9 aa, synthetic construct
GGSGRDHID

SEQ ID NO: 35499 - protein, 9 aa, synthetic construct
GGSGRDHIV

SEQ ID NO: 35500 - protein, 9 aa, synthetic construct
GGSGRDHLK

SEQ ID NO: 35501 - protein, 9 aa, synthetic construct
GGSGRDIAL

SEQ ID NO: 35502 - protein, 9 aa, synthetic construct
GGSGRDIFI

SEQ ID NO: 35503 - protein, 9 aa, synthetic construct
GGSGRDIID

SEQ ID NO: 35504 - protein, 9 aa, synthetic construct
GGSGRDILF

SEQ ID NO: 35505 - protein, 9 aa, synthetic construct
GGSGRDILM

SEQ ID NO: 35506 - protein, 9 aa, synthetic construct
GGSGRDILS

SEQ ID NO: 35507 - protein, 9 aa, synthetic construct
GGSGRDILV

SEQ ID NO: 35508 - protein, 9 aa, synthetic construct
GGSGRDIMT

SEQ ID NO: 35509 - protein, 9 aa, synthetic construct
GGSGRDIVL

SEQ ID NO: 35510 - protein, 9 aa, synthetic construct
GGSGRDIVS

SEQ ID NO: 35511 - protein, 9 aa, synthetic construct
GGSGRDKID

SEQ ID NO: 35512 - protein, 9 aa, synthetic construct
GGSGRDKMS

SEQ ID NO: 35513 - protein, 9 aa, synthetic construct
GGSGRDKMT

SEQ ID NO: 35514 - protein, 9 aa, synthetic construct
GGSGRDLAF

SEQ ID NO: 35515 - protein, 9 aa, synthetic construct
GGSGRDLAV

SEQ ID NO: 35516 - protein, 9 aa, synthetic construct
GGSGRDEMT

SEQ ID NO: 35517 - protein, 9 aa, synthetic construct
GGSGRDEMH

SEQ ID NO: 35518 - protein, 9 aa, synthetic construct
GGSGRDELD

SEQ ID NO: 35519 - protein, 9 aa, synthetic construct
GGSGRDAIG

SEQ ID NO: 35520 - protein, 9 aa, synthetic construct
GGSGQDVFQ

SEQ ID NO: 35521 - protein, 9 aa, synthetic construct
GGSGQDVFR

SEQ ID NO: 35522 - protein, 9 aa, synthetic construct
GGSGQDVFS

SEQ ID NO: 35523 - protein, 9 aa, synthetic construct
GGSGQDVIM

SEQ ID NO: 35524 - protein, 9 aa, synthetic construct
GGSGQDVIS

SEQ ID NO: 35525 - protein, 9 aa, synthetic construct
GGSGQDVLM

SEQ ID NO: 35526 - protein, 9 aa, synthetic construct
GGSGQDVLY

SEQ ID NO: 35527 - protein, 9 aa, synthetic construct
GGSGQDWAD

SEQ ID NO: 35528 - protein, 9 aa, synthetic construct
GGSGQDWMF

SEQ ID NO: 35529 - protein, 9 aa, synthetic construct
GGSGQDYID

SEQ ID NO: 35530 - protein, 9 aa, synthetic construct
GGSGQDYLE

SEQ ID NO: 35531 - protein, 9 aa, synthetic construct
GGSGRDAFR

SEQ ID NO: 35532 - protein, 9 aa, synthetic construct
GGSGRDAFT

SEQ ID NO: 35533 - protein, 9 aa, synthetic construct
GGSGRDALE

SEQ ID NO: 35534 - protein, 9 aa, synthetic construct
GGSGRDEIW

SEQ ID NO: 35535 - protein, 9 aa, synthetic construct
GGSGRDALH

SEQ ID NO: 35536 - protein, 9 aa, synthetic construct
GGSGRDALS

SEQ ID NO: 35537 - protein, 9 aa, synthetic construct
GGSGRDALT

SEQ ID NO: 35538 - protein, 9 aa, synthetic construct
GGSGRDAMS

SEQ ID NO: 35539 - protein, 9 aa, synthetic construct
GGSGRDDIF

SEQ ID NO: 35540 - protein, 9 aa, synthetic construct
GGSGRDDLA

SEQ ID NO: 35541 - protein, 9 aa, synthetic construct
GGSGRDDLE

SEQ ID NO: 35542 - protein, 9 aa, synthetic construct
GGSGRDDLF

SEQ ID NO: 35543 - protein, 9 aa, synthetic construct
GGSGRDDLQ

SEQ ID NO: 35544 - protein, 9 aa, synthetic construct
GGSGRDDLY

SEQ ID NO: 35545 - protein, 9 aa, synthetic construct
GGSGRDDMY

SEQ ID NO: 35546 - protein, 9 aa, synthetic construct
GGSGRDDVR

SEQ ID NO: 35547 - protein, 9 aa, synthetic construct
GGSGRDEFT

SEQ ID NO: 35548 - protein, 9 aa, synthetic construct
GGSGQDAFL

SEQ ID NO: 35549 - protein, 9 aa, synthetic construct
GGSGPDVLH

SEQ ID NO: 35550 - protein, 9 aa, synthetic construct
GGSGPDVFV

SEQ ID NO: 35551 - protein, 9 aa, synthetic construct
GGSGPDTMT

SEQ ID NO: 35552 - protein, 9 aa, synthetic construct
GGSGNDTAN

SEQ ID NO: 35553 - protein, 9 aa, synthetic construct
GGSGNDTFQ

SEQ ID NO: 35554 - protein, 9 aa, synthetic construct
GGSGNDTIW

SEQ ID NO: 35555 - protein, 9 aa, synthetic construct
GGSGNDTMG

SEQ ID NO: 35556 - protein, 9 aa, synthetic construct
GGSGNDTMK

SEQ ID NO: 35557 - protein, 9 aa, synthetic construct
GGSGNDTMN

SEQ ID NO: 35558 - protein, 9 aa, synthetic construct
GGSGNDTVG

SEQ ID NO: 35559 - protein, 9 aa, synthetic construct
GGSGNDTVK

SEQ ID NO: 35560 - protein, 9 aa, synthetic construct
GGSGNDTYD

SEQ ID NO: 35561 - protein, 9 aa, synthetic construct
GGSGNDTYE

SEQ ID NO: 35562 - protein, 9 aa, synthetic construct
GGSGNDTYM

SEQ ID NO: 35563 - protein, 9 aa, synthetic construct
GGSGNDTYS

SEQ ID NO: 35564 - protein, 9 aa, synthetic construct
GGSGNDTYW

SEQ ID NO: 35565 - protein, 9 aa, synthetic construct
GGSGNDVAA

SEQ ID NO: 35566 - protein, 9 aa, synthetic construct
GGSGNDVAH

SEQ ID NO: 35567 - protein, 9 aa, synthetic construct
GGSGNDVFL

SEQ ID NO: 35568 - protein, 9 aa, synthetic construct
GGSGNDVFN

SEQ ID NO: 35569 - protein, 9 aa, synthetic construct
GGSGNDVFT

SEQ ID NO: 35570 - protein, 9 aa, synthetic construct
GGSGNDVFW

SEQ ID NO: 35571 - protein, 9 aa, synthetic construct
GGSGNDVIK

SEQ ID NO: 35572 - protein, 9 aa, synthetic construct
GGSGNDVLC

SEQ ID NO: 35573 - protein, 9 aa, synthetic construct
GGSGNDVMA

SEQ ID NO: 35574 - protein, 9 aa, synthetic construct
GGSGNDVME

SEQ ID NO: 35575 - protein, 9 aa, synthetic construct
GGSGNDVMF

SEQ ID NO: 35576 - protein, 9 aa, synthetic construct
GGSGNDVMY

SEQ ID NO: 35577 - protein, 9 aa, synthetic construct
GGSGNDVVF

SEQ ID NO: 35578 - protein, 9 aa, synthetic construct
GGSGNDVVG

SEQ ID NO: 35579 - protein, 9 aa, synthetic construct
GGSGNDVVH

SEQ ID NO: 35580 - protein, 9 aa, synthetic construct
GGSGNDVVN

SEQ ID NO: 35581 - protein, 9 aa, synthetic construct
GGSGNDTAG

SEQ ID NO: 35582 - protein, 9 aa, synthetic construct
GGSGNDTAF

SEQ ID NO: 35583 - protein, 9 aa, synthetic construct
GGSGNDTAE

SEQ ID NO: 35584 - protein, 9 aa, synthetic construct
GGSGNDRVV

SEQ ID NO: 35585 - protein, 9 aa, synthetic construct
GGSGNDRFY

SEQ ID NO: 35586 - protein, 9 aa, synthetic construct
GGSGNDRIH

SEQ ID NO: 35587 - protein, 9 aa, synthetic construct
GGSGNDRIK

SEQ ID NO: 35588 - protein, 9 aa, synthetic construct
GGSGNDRIL

SEQ ID NO: 35589 - protein, 9 aa, synthetic construct
GGSGNDRIM

SEQ ID NO: 35590 - protein, 9 aa, synthetic construct
GGSGNDRMA

SEQ ID NO: 35591 - protein, 9 aa, synthetic construct
GGSGNDRMG

SEQ ID NO: 35592 - protein, 9 aa, synthetic construct
GGSGNDRMI

SEQ ID NO: 35593 - protein, 9 aa, synthetic construct
GGSGNDRMM

SEQ ID NO: 35594 - protein, 9 aa, synthetic construct
GGSGNDRMN

SEQ ID NO: 35595 - protein, 9 aa, synthetic construct
GGSGNDRMR

SEQ ID NO: 35596 - protein, 9 aa, synthetic construct
GGSGNDRVF

SEQ ID NO: 35597 - protein, 9 aa, synthetic construct
GGSGNDRVQ

SEQ ID NO: 35598 - protein, 9 aa, synthetic construct
GGSGNDRYF

SEQ ID NO: 35599 - protein, 9 aa, synthetic construct
GGSGNDSYY

SEQ ID NO: 35600 - protein, 9 aa, synthetic construct
GGSGNDRYY

SEQ ID NO: 35601 - protein, 9 aa, synthetic construct
GGSGNDSAY

SEQ ID NO: 35602 - protein, 9 aa, synthetic construct
GGSGNDSFR

SEQ ID NO: 35603 - protein, 9 aa, synthetic construct
GGSGNDSFS

SEQ ID NO: 35604 - protein, 9 aa, synthetic construct
GGSGNDSFT

SEQ ID NO: 35605 - protein, 9 aa, synthetic construct
GGSGNDSFY

SEQ ID NO: 35606 - protein, 9 aa, synthetic construct
GGSGNDSIH

SEQ ID NO: 35607 - protein, 9 aa, synthetic construct
GGSGNDSIR

SEQ ID NO: 35608 - protein, 9 aa, synthetic construct
GGSGNDSLH

SEQ ID NO: 35609 - protein, 9 aa, synthetic construct
GGSGNDSMH

SEQ ID NO: 35610 - protein, 9 aa, synthetic construct
GGSGNDSMQ

SEQ ID NO: 35611 - protein, 9 aa, synthetic construct
GGSGNDSVI

SEQ ID NO: 35612 - protein, 9 aa, synthetic construct
GGSGNDSVR

SEQ ID NO: 35613 - protein, 9 aa, synthetic construct
GGSGNDVVR

SEQ ID NO: 35614 - protein, 9 aa, synthetic construct
GGSGNDVYA

SEQ ID NO: 35615 - protein, 9 aa, synthetic construct
GGSGNDWAT

SEQ ID NO: 35616 - protein, 9 aa, synthetic construct
GGSGPDRFL

SEQ ID NO: 35617 - protein, 9 aa, synthetic construct
GGSGNDYYY

SEQ ID NO: 35618 - protein, 9 aa, synthetic construct
GGSGPDALH

SEQ ID NO: 35619 - protein, 9 aa, synthetic construct
GGSGPDALI

SEQ ID NO: 35620 - protein, 9 aa, synthetic construct
GGSGPDFLI

SEQ ID NO: 35621 - protein, 9 aa, synthetic construct
GGSGPDIFV

SEQ ID NO: 35622 - protein, 9 aa, synthetic construct
GGSGPDILL

SEQ ID NO: 35623 - protein, 9 aa, synthetic construct
GGSGPDLIW

SEQ ID NO: 35624 - protein, 9 aa, synthetic construct
GGSGPDLLK

SEQ ID NO: 35625 - protein, 9 aa, synthetic construct
GGSGPDLLV

SEQ ID NO: 35626 - protein, 9 aa, synthetic construct
GGSGPDLVL

SEQ ID NO: 35627 - protein, 9 aa, synthetic construct
GGSGPDNLF

SEQ ID NO: 35628 - protein, 9 aa, synthetic construct
GGSGPDQFI

SEQ ID NO: 35629 - protein, 9 aa, synthetic construct
GGSGPDQIS

SEQ ID NO: 35630 - protein, 9 aa, synthetic construct
GGSGPDRIF

SEQ ID NO: 35631 - protein, 9 aa, synthetic construct
GGSGNDYVK

SEQ ID NO: 35632 - protein, 9 aa, synthetic construct
GGSGPDRIN

SEQ ID NO: 35633 - protein, 9 aa, synthetic construct
GGSGPDRLE

SEQ ID NO: 35634 - protein, 9 aa, synthetic construct
GGSGPDRLF

SEQ ID NO: 35635 - protein, 9 aa, synthetic construct
GGSGPDRMS

SEQ ID NO: 35636 - protein, 9 aa, synthetic construct
GGSGPDRMT

SEQ ID NO: 35637 - protein, 9 aa, synthetic construct
GGSGPDSLL

SEQ ID NO: 35638 - protein, 9 aa, synthetic construct
GGSGPDTFM

SEQ ID NO: 35639 - protein, 9 aa, synthetic construct
GGSGPDTII

SEQ ID NO: 35640 - protein, 9 aa, synthetic construct
GGSGPDTLA

SEQ ID NO: 35641 - protein, 9 aa, synthetic construct
GGSGPDTLD

SEQ ID NO: 35642 - protein, 9 aa, synthetic construct
GGSGPDTLQ

SEQ ID NO: 35643 - protein, 9 aa, synthetic construct
GGSGPDTLS

SEQ ID NO: 35644 - protein, 9 aa, synthetic construct
GGSGPDTLW

SEQ ID NO: 35645 - protein, 9 aa, synthetic construct
GGSGNDYVV

SEQ ID NO: 35646 - protein, 9 aa, synthetic construct
GGSGNDYMV

SEQ ID NO: 35647 - protein, 9 aa, synthetic construct
GGSGNDWIA

SEQ ID NO: 35648 - protein, 9 aa, synthetic construct
GGSGNDYAD

SEQ ID NO: 35649 - protein, 9 aa, synthetic construct
GGSGNDWIV

SEQ ID NO: 35650 - protein, 9 aa, synthetic construct
GGSGNDWIW

SEQ ID NO: 35651 - protein, 9 aa, synthetic construct
GGSGNDWIY

SEQ ID NO: 35652 - protein, 9 aa, synthetic construct
GGSGNDWLG

SEQ ID NO: 35653 - protein, 9 aa, synthetic construct
GGSGNDWLR

SEQ ID NO: 35654 - protein, 9 aa, synthetic construct
GGSGNDWLV

SEQ ID NO: 35655 - protein, 9 aa, synthetic construct
GGSGNDWME

SEQ ID NO: 35656 - protein, 9 aa, synthetic construct
GGSGNDWMK

SEQ ID NO: 35657 - protein, 9 aa, synthetic construct
GGSGNDWVA

SEQ ID NO: 35658 - protein, 9 aa, synthetic construct
GGSGNDWVN

SEQ ID NO: 35659 - protein, 9 aa, synthetic construct
GGSGNDWVS

SEQ ID NO: 35660 - protein, 9 aa, synthetic construct
GGSGNDWVV

SEQ ID NO: 35661 - protein, 9 aa, synthetic construct
GGSGNDXLF

SEQ ID NO: 35662 - protein, 9 aa, synthetic construct
GGSGNDYAN

SEQ ID NO: 35663 - protein, 9 aa, synthetic construct
GGSGNDYMN

SEQ ID NO: 35664 - protein, 9 aa, synthetic construct
GGSGNDYAW

SEQ ID NO: 35665 - protein, 9 aa, synthetic construct
GGSGNDYFF

SEQ ID NO: 35666 - protein, 9 aa, synthetic construct
GGSGNDYFV

SEQ ID NO: 35667 - protein, 9 aa, synthetic construct
GGSGNDYFY

SEQ ID NO: 35668 - protein, 9 aa, synthetic construct
GGSGNDYII

SEQ ID NO: 35669 - protein, 9 aa, synthetic construct
GGSGNDYIL

SEQ ID NO: 35670 - protein, 9 aa, synthetic construct
GGSGNDYIM

SEQ ID NO: 35671 - protein, 9 aa, synthetic construct
GGSGNDYIN

SEQ ID NO: 35672 - protein, 9 aa, synthetic construct
GGSGNDYIQ

SEQ ID NO: 35673 - protein, 9 aa, synthetic construct
GGSGNDYIV

SEQ ID NO: 35674 - protein, 9 aa, synthetic construct
GGSGNDYLG

SEQ ID NO: 35675 - protein, 9 aa, synthetic construct
GGSGNDYLH

SEQ ID NO: 35676 - protein, 9 aa, synthetic construct
GGSGNDYLQ

SEQ ID NO: 35677 - protein, 9 aa, synthetic construct
GGSGLDKLF

SEQ ID NO: 35678 - protein, 9 aa, synthetic construct
GGSGLDIVD

SEQ ID NO: 35679 - protein, 9 aa, synthetic construct
GGSGLDILY

SEQ ID NO: 35680 - protein, 9 aa, synthetic construct
GGSGGDSLD

SEQ ID NO: 35681 - protein, 9 aa, synthetic construct
GGSGGDLLE

SEQ ID NO: 35682 - protein, 9 aa, synthetic construct
GGSGGDLLG

SEQ ID NO: 35683 - protein, 9 aa, synthetic construct
GGSGGDLLI

SEQ ID NO: 35684 - protein, 9 aa, synthetic construct
GGSGGDLLK

SEQ ID NO: 35685 - protein, 9 aa, synthetic construct
GGSGGDLLY

SEQ ID NO: 35686 - protein, 9 aa, synthetic construct
GGSGGDLME

SEQ ID NO: 35687 - protein, 9 aa, synthetic construct
GGSGGDLMF

SEQ ID NO: 35688 - protein, 9 aa, synthetic construct
GGSGGDLMK

SEQ ID NO: 35689 - protein, 9 aa, synthetic construct
GGSGGDLVY

SEQ ID NO: 35690 - protein, 9 aa, synthetic construct
GGSGGDMLF

SEQ ID NO: 35691 - protein, 9 aa, synthetic construct
GGSGGDNLL

SEQ ID NO: 35692 - protein, 9 aa, synthetic construct
GGSGGDNLN

SEQ ID NO: 35693 - protein, 9 aa, synthetic construct
GGSGGDQFI

SEQ ID NO: 35694 - protein, 9 aa, synthetic construct
GGSGGDQFR

SEQ ID NO: 35695 - protein, 9 aa, synthetic construct
GGSGGDQIS

SEQ ID NO: 35696 - protein, 9 aa, synthetic construct
GGSGGDQLT

SEQ ID NO: 35697 - protein, 9 aa, synthetic construct
GGSGGDQVS

SEQ ID NO: 35698 - protein, 9 aa, synthetic construct
GGSGGDRFY

SEQ ID NO: 35699 - protein, 9 aa, synthetic construct
GGSGGDRIN

SEQ ID NO: 35700 - protein, 9 aa, synthetic construct
GGSGGDRIW

SEQ ID NO: 35701 - protein, 9 aa, synthetic construct
GGSGGDRIY

SEQ ID NO: 35702 - protein, 9 aa, synthetic construct
GGSGGDRLD

SEQ ID NO: 35703 - protein, 9 aa, synthetic construct
GGSGGDRLI

SEQ ID NO: 35704 - protein, 9 aa, synthetic construct
GGSGGDRLN

SEQ ID NO: 35705 - protein, 9 aa, synthetic construct
GGSGGDRLT

SEQ ID NO: 35706 - protein, 9 aa, synthetic construct
GGSGGDRMD

SEQ ID NO: 35707 - protein, 9 aa, synthetic construct
GGSGGDRMT

SEQ ID NO: 35708 - protein, 9 aa, synthetic construct
GGSGGDRVW

SEQ ID NO: 35709 - protein, 9 aa, synthetic construct
GGSGGDRYY

SEQ ID NO: 35710 - protein, 9 aa, synthetic construct
GGSGGDLIY

SEQ ID NO: 35711 - protein, 9 aa, synthetic construct
GGSGGDLIT

SEQ ID NO: 35712 - protein, 9 aa, synthetic construct
GGSGGDLFI

SEQ ID NO: 35713 - protein, 9 aa, synthetic construct
GGSGGDHLH

SEQ ID NO: 35714 - protein, 9 aa, synthetic construct
GGSGGDDYD

SEQ ID NO: 35715 - protein, 9 aa, synthetic construct
GGSGGDEFQ

SEQ ID NO: 35716 - protein, 9 aa, synthetic construct
GGSGGDEIR

SEQ ID NO: 35717 - protein, 9 aa, synthetic construct
GGSGGDELA

SEQ ID NO: 35718 - protein, 9 aa, synthetic construct
GGSGGDELF

SEQ ID NO: 35719 - protein, 9 aa, synthetic construct
GGSGGDELT

SEQ ID NO: 35720 - protein, 9 aa, synthetic construct
GGSGGDELY

SEQ ID NO: 35721 - protein, 9 aa, synthetic construct
GGSGGDFLI

SEQ ID NO: 35722 - protein, 9 aa, synthetic construct
GGSGGDFLY

SEQ ID NO: 35723 - protein, 9 aa, synthetic construct
GGSGGDFVH

SEQ ID NO: 35724 - protein, 9 aa, synthetic construct
GGSGGDFVV

SEQ ID NO: 35725 - protein, 9 aa, synthetic construct
GGSGGDGAR

SEQ ID NO: 35726 - protein, 9 aa, synthetic construct
GGSGGDHLF

SEQ ID NO: 35727 - protein, 9 aa, synthetic construct
GGSGGDHLL

SEQ ID NO: 35728 - protein, 9 aa, synthetic construct
GGSGGDKLY

SEQ ID NO: 35729 - protein, 9 aa, synthetic construct
GGSGGDIFA

SEQ ID NO: 35730 - protein, 9 aa, synthetic construct
GGSGGDIFD

SEQ ID NO: 35731 - protein, 9 aa, synthetic construct
GGSGGDIID

SEQ ID NO: 35732 - protein, 9 aa, synthetic construct
GGSGGDILF

SEQ ID NO: 35733 - protein, 9 aa, synthetic construct
GGSGGDILI

SEQ ID NO: 35734 - protein, 9 aa, synthetic construct
GGSGGDILL

SEQ ID NO: 35735 - protein, 9 aa, synthetic construct
GGSGGDILN

SEQ ID NO: 35736 - protein, 9 aa, synthetic construct
GGSGGDILS

SEQ ID NO: 35737 - protein, 9 aa, synthetic construct
GGSGGDILW

SEQ ID NO: 35738 - protein, 9 aa, synthetic construct
GGSGGDIMA

SEQ ID NO: 35739 - protein, 9 aa, synthetic construct
GGSGGDIVM

SEQ ID NO: 35740 - protein, 9 aa, synthetic construct
GGSGGDKFV

SEQ ID NO: 35741 - protein, 9 aa, synthetic construct
GGSGGDKII

SEQ ID NO: 35742 - protein, 9 aa, synthetic construct
GGSGGDSIN

SEQ ID NO: 35743 - protein, 9 aa, synthetic construct
GGSGGDSLE

SEQ ID NO: 35744 - protein, 9 aa, synthetic construct
GGSGLDILN

SEQ ID NO: 35745 - protein, 9 aa, synthetic construct
GGSGGDSLK

SEQ ID NO: 35746 - protein, 9 aa, synthetic construct
GGSGGDYIE

SEQ ID NO: 35747 - protein, 9 aa, synthetic construct
GGSGGDYLI

SEQ ID NO: 35748 - protein, 9 aa, synthetic construct
GGSGGDYLS

SEQ ID NO: 35749 - protein, 9 aa, synthetic construct
GGSGGDYLT

SEQ ID NO: 35750 - protein, 9 aa, synthetic construct
GGSGGDYMW

SEQ ID NO: 35751 - protein, 9 aa, synthetic construct
GGSGHDAFI

SEQ ID NO: 35752 - protein, 9 aa, synthetic construct
GGSGHDAIF

SEQ ID NO: 35753 - protein, 9 aa, synthetic construct
GGSGHDALL

SEQ ID NO: 35754 - protein, 9 aa, synthetic construct
GGSGHDALR

SEQ ID NO: 35755 - protein, 9 aa, synthetic construct
GGSGHDALW

SEQ ID NO: 35756 - protein, 9 aa, synthetic construct
GGSGHDALY

SEQ ID NO: 35757 - protein, 9 aa, synthetic construct
GGSGHDDID

SEQ ID NO: 35758 - protein, 9 aa, synthetic construct
GGSGHDDIS

SEQ ID NO: 35759 - protein, 9 aa, synthetic construct
GGSGHDDIY

SEQ ID NO: 35760 - protein, 9 aa, synthetic construct
GGSGHDDLF

SEQ ID NO: 35761 - protein, 9 aa, synthetic construct
GGSGHDDLN

SEQ ID NO: 35762 - protein, 9 aa, synthetic construct
GGSGHDDLT

SEQ ID NO: 35763 - protein, 9 aa, synthetic construct
GGSGHDDLY

SEQ ID NO: 35764 - protein, 9 aa, synthetic construct
GGSGHDEIA

SEQ ID NO: 35765 - protein, 9 aa, synthetic construct
GGSGHDEIH

SEQ ID NO: 35766 - protein, 9 aa, synthetic construct
GGSGHDEIW

SEQ ID NO: 35767 - protein, 9 aa, synthetic construct
GGSGHDELW

SEQ ID NO: 35768 - protein, 9 aa, synthetic construct
GGSGHDFIV

SEQ ID NO: 35769 - protein, 9 aa, synthetic construct
GGSGHDFLI

SEQ ID NO: 35770 - protein, 9 aa, synthetic construct
GGSGHDFVW

SEQ ID NO: 35771 - protein, 9 aa, synthetic construct
GGSGHDGLY

SEQ ID NO: 35772 - protein, 9 aa, synthetic construct
GGSGHDHLE

SEQ ID NO: 35773 - protein, 9 aa, synthetic construct
GGSGHDIAK

SEQ ID NO: 35774 - protein, 9 aa, synthetic construct
GGSGHDILD

SEQ ID NO: 35775 - protein, 9 aa, synthetic construct
GGSGGDYID

SEQ ID NO: 35776 - protein, 9 aa, synthetic construct
GGSGGDYFD

SEQ ID NO: 35777 - protein, 9 aa, synthetic construct
GGSGGDWMH

SEQ ID NO: 35778 - protein, 9 aa, synthetic construct
GGSGGDTVA

SEQ ID NO: 35779 - protein, 9 aa, synthetic construct
GGSGGDSLL

SEQ ID NO: 35780 - protein, 9 aa, synthetic construct
GGSGGDSLR

SEQ ID NO: 35781 - protein, 9 aa, synthetic construct
GGSGGDSMS

SEQ ID NO: 35782 - protein, 9 aa, synthetic construct
GGSGGDSVD

SEQ ID NO: 35783 - protein, 9 aa, synthetic construct
GGSGGDSVE

SEQ ID NO: 35784 - protein, 9 aa, synthetic construct
GGSGGDTFA

SEQ ID NO: 35785 - protein, 9 aa, synthetic construct
GGSGGDTIV

SEQ ID NO: 35786 - protein, 9 aa, synthetic construct
GGSGGDTLA

SEQ ID NO: 35787 - protein, 9 aa, synthetic construct
GGSGGDTLM

SEQ ID NO: 35788 - protein, 9 aa, synthetic construct
GGSGGDTLR

SEQ ID NO: 35789 - protein, 9 aa, synthetic construct
GGSGGDTMN

SEQ ID NO: 35790 - protein, 9 aa, synthetic construct
GGSGGDTMV

SEQ ID NO: 35791 - protein, 9 aa, synthetic construct
GGSGGDTMY

SEQ ID NO: 35792 - protein, 9 aa, synthetic construct
GGSGGDTVH

SEQ ID NO: 35793 - protein, 9 aa, synthetic construct
GGSGGDWLY

SEQ ID NO: 35794 - protein, 9 aa, synthetic construct
GGSGGDTVY

SEQ ID NO: 35795 - protein, 9 aa, synthetic construct
GGSGGDVID

SEQ ID NO: 35796 - protein, 9 aa, synthetic construct
GGSGGDVIL

SEQ ID NO: 35797 - protein, 9 aa, synthetic construct
GGSGGDVLA

SEQ ID NO: 35798 - protein, 9 aa, synthetic construct
GGSGGDVLQ

SEQ ID NO: 35799 - protein, 9 aa, synthetic construct
GGSGGDVLT

SEQ ID NO: 35800 - protein, 9 aa, synthetic construct
GGSGGDVLV

SEQ ID NO: 35801 - protein, 9 aa, synthetic construct
GGSGGDVLY

SEQ ID NO: 35802 - protein, 9 aa, synthetic construct
GGSGGDVMT

SEQ ID NO: 35803 - protein, 9 aa, synthetic construct
GGSGGDVMY

SEQ ID NO: 35804 - protein, 9 aa, synthetic construct
GGSGGDVVE

SEQ ID NO: 35805 - protein, 9 aa, synthetic construct
GGSGGDWLD

SEQ ID NO: 35806 - protein, 9 aa, synthetic construct
GGSGGDWLN

SEQ ID NO: 35807 - protein, 9 aa, synthetic construct
GGSGGDDLY

SEQ ID NO: 35808 - protein, 9 aa, synthetic construct
GGSGGDDID

SEQ ID NO: 35809 - protein, 9 aa, synthetic construct
GGSGGDDFL

SEQ ID NO: 35810 - protein, 9 aa, synthetic construct
GGSGGDAYA

SEQ ID NO: 35811 - protein, 9 aa, synthetic construct
GGSGEDSVD

SEQ ID NO: 35812 - protein, 9 aa, synthetic construct
GGSGEDSVK

SEQ ID NO: 35813 - protein, 9 aa, synthetic construct
GGSGEDTAT

SEQ ID NO: 35814 - protein, 9 aa, synthetic construct
GGSGEDTFD

SEQ ID NO: 35815 - protein, 9 aa, synthetic construct
GGSGEDTFI

SEQ ID NO: 35816 - protein, 9 aa, synthetic construct
GGSGEDTIE

SEQ ID NO: 35817 - protein, 9 aa, synthetic construct
GGSGEDTIG

SEQ ID NO: 35818 - protein, 9 aa, synthetic construct
GGSGEDTII

SEQ ID NO: 35819 - protein, 9 aa, synthetic construct
GGSGEDTIT

SEQ ID NO: 35820 - protein, 9 aa, synthetic construct
GGSGEDTLA

SEQ ID NO: 35821 - protein, 9 aa, synthetic construct
GGSGEDTLF

SEQ ID NO: 35822 - protein, 9 aa, synthetic construct
GGSGEDTLH

SEQ ID NO: 35823 - protein, 9 aa, synthetic construct
GGSGEDTLM

SEQ ID NO: 35824 - protein, 9 aa, synthetic construct
GGSGEDTLS

SEQ ID NO: 35825 - protein, 9 aa, synthetic construct
GGSGEDTMT

SEQ ID NO: 35826 - protein, 9 aa, synthetic construct
GGSGEDTVI

SEQ ID NO: 35827 - protein, 9 aa, synthetic construct
GGSGEDVIV

SEQ ID NO: 35828 - protein, 9 aa, synthetic construct
GGSGEDVLK

SEQ ID NO: 35829 - protein, 9 aa, synthetic construct
GGSGEDVLN

SEQ ID NO: 35830 - protein, 9 aa, synthetic construct
GGSGEDVLS

SEQ ID NO: 35831 - protein, 9 aa, synthetic construct
GGSGEDWFV

SEQ ID NO: 35832 - protein, 9 aa, synthetic construct
GGSGEDWIL

SEQ ID NO: 35833 - protein, 9 aa, synthetic construct
GGSGEDYID

SEQ ID NO: 35834 - protein, 9 aa, synthetic construct
GGSGEDYLY

SEQ ID NO: 35835 - protein, 9 aa, synthetic construct
GGSGFDAAT

SEQ ID NO: 35836 - protein, 9 aa, synthetic construct
GGSGFDALS

SEQ ID NO: 35837 - protein, 9 aa, synthetic construct
GGSGFDDIN

SEQ ID NO: 35838 - protein, 9 aa, synthetic construct
GGSGFDDIY

SEQ ID NO: 35839 - protein, 9 aa, synthetic construct
GGSGFDDLD

SEQ ID NO: 35840 - protein, 9 aa, synthetic construct
GGSGEDSLM

SEQ ID NO: 35841 - protein, 9 aa, synthetic construct
GGSGEDSLL

SEQ ID NO: 35842 - protein, 9 aa, synthetic construct
GGSGEDSLH

SEQ ID NO: 35843 - protein, 9 aa, synthetic construct
GGSGEDQLD

SEQ ID NO: 35844 - protein, 9 aa, synthetic construct
GGSGEDILT

SEQ ID NO: 35845 - protein, 9 aa, synthetic construct
GGSGEDIML

SEQ ID NO: 35846 - protein, 9 aa, synthetic construct
GGSGEDKAF

SEQ ID NO: 35847 - protein, 9 aa, synthetic construct
GGSGEDKID

SEQ ID NO: 35848 - protein, 9 aa, synthetic construct
GGSGEDKLN

SEQ ID NO: 35849 - protein, 9 aa, synthetic construct
GGSGEDKLW

SEQ ID NO: 35850 - protein, 9 aa, synthetic construct
GGSGEDKMS

SEQ ID NO: 35851 - protein, 9 aa, synthetic construct
GGSGEDLFX

SEQ ID NO: 35852 - protein, 9 aa, synthetic construct
GGSGEDLMY

SEQ ID NO: 35853 - protein, 9 aa, synthetic construct
GGSGEDMFV

SEQ ID NO: 35854 - protein, 9 aa, synthetic construct
GGSGEDMLN

SEQ ID NO: 35855 - protein, 9 aa, synthetic construct
GGSGEDMLY

SEQ ID NO: 35856 - protein, 9 aa, synthetic construct
GGSGEDMVL

SEQ ID NO: 35857 - protein, 9 aa, synthetic construct
GGSGEDQLL

SEQ ID NO: 35858 - protein, 9 aa, synthetic construct
GGSGEDSLD

SEQ ID NO: 35859 - protein, 9 aa, synthetic construct
GGSGEDQLR

SEQ ID NO: 35860 - protein, 9 aa, synthetic construct
GGSGEDQLS

SEQ ID NO: 35861 - protein, 9 aa, synthetic construct
GGSGEDRFD

SEQ ID NO: 35862 - protein, 9 aa, synthetic construct
GGSGEDRFV

SEQ ID NO: 35863 - protein, 9 aa, synthetic construct
GGSGEDRLD

SEQ ID NO: 35864 - protein, 9 aa, synthetic construct
GGSGEDRLE

SEQ ID NO: 35865 - protein, 9 aa, synthetic construct
GGSGEDRVA

SEQ ID NO: 35866 - protein, 9 aa, synthetic construct
GGSGEDSFL

SEQ ID NO: 35867 - protein, 9 aa, synthetic construct
GGSGEDSFV

SEQ ID NO: 35868 - protein, 9 aa, synthetic construct
GGSGEDSIE

SEQ ID NO: 35869 - protein, 9 aa, synthetic construct
GGSGEDSII

SEQ ID NO: 35870 - protein, 9 aa, synthetic construct
GGSGEDSIT

SEQ ID NO: 35871 - protein, 9 aa, synthetic construct
GGSGEDSIV

SEQ ID NO: 35872 - protein, 9 aa, synthetic construct
GGSGFDDLH

SEQ ID NO: 35873 - protein, 9 aa, synthetic construct
GGSGFDDLK

SEQ ID NO: 35874 - protein, 9 aa, synthetic construct
GGSGFDDVS

SEQ ID NO: 35875 - protein, 9 aa, synthetic construct
GGSGFDVLS

SEQ ID NO: 35876 - protein, 9 aa, synthetic construct
GGSGFDTIN

SEQ ID NO: 35877 - protein, 9 aa, synthetic construct
GGSGFDTIY

SEQ ID NO: 35878 - protein, 9 aa, synthetic construct
GGSGFDTLF

SEQ ID NO: 35879 - protein, 9 aa, synthetic construct
GGSGFDTLL

SEQ ID NO: 35880 - protein, 9 aa, synthetic construct
GGSGFDTLN

SEQ ID NO: 35881 - protein, 9 aa, synthetic construct
GGSGFDTLT

SEQ ID NO: 35882 - protein, 9 aa, synthetic construct
GGSGFDTLY

SEQ ID NO: 35883 - protein, 9 aa, synthetic construct
GGSGFDTMH

SEQ ID NO: 35884 - protein, 9 aa, synthetic construct
GGSGFDTMI

SEQ ID NO: 35885 - protein, 9 aa, synthetic construct
GGSGFDVAD

SEQ ID NO: 35886 - protein, 9 aa, synthetic construct
GGSGFDVID

SEQ ID NO: 35887 - protein, 9 aa, synthetic construct
GGSGFDVLD

SEQ ID NO: 35888 - protein, 9 aa, synthetic construct
GGSGFDVLF

SEQ ID NO: 35889 - protein, 9 aa, synthetic construct
GGSGFDVLT

SEQ ID NO: 35890 - protein, 9 aa, synthetic construct
GGSGFDTIE

SEQ ID NO: 35891 - protein, 9 aa, synthetic construct
GGSGFDVLV

SEQ ID NO: 35892 - protein, 9 aa, synthetic construct
GGSGFDVVD

SEQ ID NO: 35893 - protein, 9 aa, synthetic construct
GGSGFDVYF

SEQ ID NO: 35894 - protein, 9 aa, synthetic construct
GGSGFDWLQ

SEQ ID NO: 35895 - protein, 9 aa, synthetic construct
GGSGFDYAS

SEQ ID NO: 35896 - protein, 9 aa, synthetic construct
GGSGFDYLD

SEQ ID NO: 35897 - protein, 9 aa, synthetic construct
GGSGFDYVR

SEQ ID NO: 35898 - protein, 9 aa, synthetic construct
GGSGGDAFC

SEQ ID NO: 35899 - protein, 9 aa, synthetic construct
GGSGGDAFI

SEQ ID NO: 35900 - protein, 9 aa, synthetic construct
GGSGGDAIF

SEQ ID NO: 35901 - protein, 9 aa, synthetic construct
GGSGGDAIH

SEQ ID NO: 35902 - protein, 9 aa, synthetic construct
GGSGGDALD

SEQ ID NO: 35903 - protein, 9 aa, synthetic construct
GGSGGDAME

SEQ ID NO: 35904 - protein, 9 aa, synthetic construct
GGSGFDTII

SEQ ID NO: 35905 - protein, 9 aa, synthetic construct
GGSGFDTID

SEQ ID NO: 35906 - protein, 9 aa, synthetic construct
GGSGFDEIS

SEQ ID NO: 35907 - protein, 9 aa, synthetic construct
GGSGFDNIH

SEQ ID NO: 35908 - protein, 9 aa, synthetic construct
GGSGFDEIW

SEQ ID NO: 35909 - protein, 9 aa, synthetic construct
GGSGFDELH

SEQ ID NO: 35910 - protein, 9 aa, synthetic construct
GGSGFDFAH

SEQ ID NO: 35911 - protein, 9 aa, synthetic construct
GGSGFDFLI

SEQ ID NO: 35912 - protein, 9 aa, synthetic construct
GGSGFDHLF

SEQ ID NO: 35913 - protein, 9 aa, synthetic construct
GGSGFDIMY

SEQ ID NO: 35914 - protein, 9 aa, synthetic construct
GGSGFDIYD

SEQ ID NO: 35915 - protein, 9 aa, synthetic construct
GGSGFDKLT

SEQ ID NO: 35916 - protein, 9 aa, synthetic construct
GGSGFDLIT

SEQ ID NO: 35917 - protein, 9 aa, synthetic construct
GGSGFDLLF

SEQ ID NO: 35918 - protein, 9 aa, synthetic construct
GGSGFDMAI

SEQ ID NO: 35919 - protein, 9 aa, synthetic construct
GGSGFDMLT

SEQ ID NO: 35920 - protein, 9 aa, synthetic construct
GGSGFDNFV

SEQ ID NO: 35921 - protein, 9 aa, synthetic construct
GGSGFDNLF

SEQ ID NO: 35922 - protein, 9 aa, synthetic construct
GGSGFDTAY

SEQ ID NO: 35923 - protein, 9 aa, synthetic construct
GGSGFDNLN

SEQ ID NO: 35924 - protein, 9 aa, synthetic construct
GGSGFDQAT

SEQ ID NO: 35925 - protein, 9 aa, synthetic construct
GGSGFDQID

SEQ ID NO: 35926 - protein, 9 aa, synthetic construct
GGSGFDQLF

SEQ ID NO: 35927 - protein, 9 aa, synthetic construct
GGSGFDQMD

SEQ ID NO: 35928 - protein, 9 aa, synthetic construct
GGSGFDRLE

SEQ ID NO: 35929 - protein, 9 aa, synthetic construct
GGSGFDRLY

SEQ ID NO: 35930 - protein, 9 aa, synthetic construct
GGSGFDRMD

SEQ ID NO: 35931 - protein, 9 aa, synthetic construct
GGSGFDSAM

SEQ ID NO: 35932 - protein, 9 aa, synthetic construct
GGSGFDSLN

SEQ ID NO: 35933 - protein, 9 aa, synthetic construct
GGSGFDSLS

SEQ ID NO: 35934 - protein, 9 aa, synthetic construct
GGSGFDTAD

SEQ ID NO: 35935 - protein, 9 aa, synthetic construct
GGSGFDTAS

SEQ ID NO: 35936 - protein, 9 aa, synthetic construct
GGSGHDILK

SEQ ID NO: 35937 - protein, 9 aa, synthetic construct
GGSGHDILP

SEQ ID NO: 35938 - protein, 9 aa, synthetic construct
GGSGHDILR

SEQ ID NO: 35939 - protein, 9 aa, synthetic construct
GGSGIDSIV

SEQ ID NO: 35940 - protein, 9 aa, synthetic construct
GGSGIDWMD

SEQ ID NO: 35941 - protein, 9 aa, synthetic construct
GGSGIDYIS

SEQ ID NO: 35942 - protein, 9 aa, synthetic construct
GGSGIDYLS

SEQ ID NO: 35943 - protein, 9 aa, synthetic construct
GGSGKDAFR

SEQ ID NO: 35944 - protein, 9 aa, synthetic construct
GGSGKDALF

SEQ ID NO: 35945 - protein, 9 aa, synthetic construct
GGSGKDAMV

SEQ ID NO: 35946 - protein, 9 aa, synthetic construct
GGSGKDDLR

SEQ ID NO: 35947 - protein, 9 aa, synthetic construct
GGSGKDDVH

SEQ ID NO: 35948 - protein, 9 aa, synthetic construct
GGSGKDEIR

SEQ ID NO: 35949 - protein, 9 aa, synthetic construct
GGSGKDELD

SEQ ID NO: 35950 - protein, 9 aa, synthetic construct
GGSGKDELK

SEQ ID NO: 35951 - protein, 9 aa, synthetic construct
GGSGKDFLI

SEQ ID NO: 35952 - protein, 9 aa, synthetic construct
GGSGKDFLS

SEQ ID NO: 35953 - protein, 9 aa, synthetic construct
GGSGKDGLF

SEQ ID NO: 35954 - protein, 9 aa, synthetic construct
GGSGKDGVY

SEQ ID NO: 35955 - protein, 9 aa, synthetic construct
GGSGKDHMS

SEQ ID NO: 35956 - protein, 9 aa, synthetic construct
GGSGKDIFG

SEQ ID NO: 35957 - protein, 9 aa, synthetic construct
GGSGKDIFM

SEQ ID NO: 35958 - protein, 9 aa, synthetic construct
GGSGKDIIK

SEQ ID NO: 35959 - protein, 9 aa, synthetic construct
GGSGKDIIS

SEQ ID NO: 35960 - protein, 9 aa, synthetic construct
GGSGKDILE

SEQ ID NO: 35961 - protein, 9 aa, synthetic construct
GGSGKDILS

SEQ ID NO: 35962 - protein, 9 aa, synthetic construct
GGSGKDILT

SEQ ID NO: 35963 - protein, 9 aa, synthetic construct
GGSGKDILV

SEQ ID NO: 35964 - protein, 9 aa, synthetic construct
GGSGKDKAR

SEQ ID NO: 35965 - protein, 9 aa, synthetic construct
GGSGKDKFI

SEQ ID NO: 35966 - protein, 9 aa, synthetic construct
GGSGKDKIN

SEQ ID NO: 35967 - protein, 9 aa, synthetic construct
GGSGKDKIY

SEQ ID NO: 35968 - protein, 9 aa, synthetic construct
GGSGKDKLL

SEQ ID NO: 35969 - protein, 9 aa, synthetic construct
GGSGIDWAS

SEQ ID NO: 35970 - protein, 9 aa, synthetic construct
GGSGIDVVS

SEQ ID NO: 35971 - protein, 9 aa, synthetic construct
GGSGIDVVD

SEQ ID NO: 35972 - protein, 9 aa, synthetic construct
GGSGIDTLL

SEQ ID NO: 35973 - protein, 9 aa, synthetic construct
GGSGIDSLL

SEQ ID NO: 35974 - protein, 9 aa, synthetic construct
GGSGIDSLR

SEQ ID NO: 35975 - protein, 9 aa, synthetic construct
GGSGIDTAK

SEQ ID NO: 35976 - protein, 9 aa, synthetic construct
GGSGIDTAL

SEQ ID NO: 35977 - protein, 9 aa, synthetic construct
GGSGIDTAN

SEQ ID NO: 35978 - protein, 9 aa, synthetic construct
GGSGIDTAT

SEQ ID NO: 35979 - protein, 9 aa, synthetic construct
GGSGIDTFK

SEQ ID NO: 35980 - protein, 9 aa, synthetic construct
GGSGIDTFL

SEQ ID NO: 35981 - protein, 9 aa, synthetic construct
GGSGIDTID

SEQ ID NO: 35982 - protein, 9 aa, synthetic construct
GGSGIDTIN

SEQ ID NO: 35983 - protein, 9 aa, synthetic construct
GGSGIDTIQ

SEQ ID NO: 35984 - protein, 9 aa, synthetic construct
GGSGIDTIS

SEQ ID NO: 35985 - protein, 9 aa, synthetic construct
GGSGIDTIT

SEQ ID NO: 35986 - protein, 9 aa, synthetic construct
GGSGIDTLQ

SEQ ID NO: 35987 - protein, 9 aa, synthetic construct
GGSGIDVLL

SEQ ID NO: 35988 - protein, 9 aa, synthetic construct
GGSGIDTMD

SEQ ID NO: 35989 - protein, 9 aa, synthetic construct
GGSGIDTMK

SEQ ID NO: 35990 - protein, 9 aa, synthetic construct
GGSGIDTMT

SEQ ID NO: 35991 - protein, 9 aa, synthetic construct
GGSGIDTMY

SEQ ID NO: 35992 - protein, 9 aa, synthetic construct
GGSGIDTVD

SEQ ID NO: 35993 - protein, 9 aa, synthetic construct
GGSGIDTVL

SEQ ID NO: 35994 - protein, 9 aa, synthetic construct
GGSGIDTVN

SEQ ID NO: 35995 - protein, 9 aa, synthetic construct
GGSGIDVAV

SEQ ID NO: 35996 - protein, 9 aa, synthetic construct
GGSGIDVID

SEQ ID NO: 35997 - protein, 9 aa, synthetic construct
GGSGIDVIF

SEQ ID NO: 35998 - protein, 9 aa, synthetic construct
GGSGIDVIH

SEQ ID NO: 35999 - protein, 9 aa, synthetic construct
GGSGIDVLD

SEQ ID NO: 36000 - protein, 9 aa, synthetic construct
GGSGIDVLI

SEQ ID NO: 36001 - protein, 9 aa, synthetic construct
GGSGKDKLT

SEQ ID NO: 36002 - protein, 9 aa, synthetic construct
GGSGKDKVM

SEQ ID NO: 36003 - protein, 9 aa, synthetic construct
GGSGKDLFK

SEQ ID NO: 36004 - protein, 9 aa, synthetic construct
GGSGLDAIA

SEQ ID NO: 36005 - protein, 9 aa, synthetic construct
GGSGKDTLM

SEQ ID NO: 36006 - protein, 9 aa, synthetic construct
GGSGKDTMF

SEQ ID NO: 36007 - protein, 9 aa, synthetic construct
GGSGKDTYV

SEQ ID NO: 36008 - protein, 9 aa, synthetic construct
GGSGKDVFI

SEQ ID NO: 36009 - protein, 9 aa, synthetic construct
GGSGKDVFQ

SEQ ID NO: 36010 - protein, 9 aa, synthetic construct
GGSGKDVIY

SEQ ID NO: 36011 - protein, 9 aa, synthetic construct
GGSGKDVLD

SEQ ID NO: 36012 - protein, 9 aa, synthetic construct
GGSGKDVVS

SEQ ID NO: 36013 - protein, 9 aa, synthetic construct
GGSGKDWLF

SEQ ID NO: 36014 - protein, 9 aa, synthetic construct
GGSGKDYID

SEQ ID NO: 36015 - protein, 9 aa, synthetic construct
GGSGKDYLA

SEQ ID NO: 36016 - protein, 9 aa, synthetic construct
GGSGKDYVD

SEQ ID NO: 36017 - protein, 9 aa, synthetic construct
GGSGKDYVE

SEQ ID NO: 36018 - protein, 9 aa, synthetic construct
GGSGLDALN

SEQ ID NO: 36019 - protein, 9 aa, synthetic construct
GGSGKDTIH

SEQ ID NO: 36020 - protein, 9 aa, synthetic construct
GGSGLDALY

SEQ ID NO: 36021 - protein, 9 aa, synthetic construct
GGSGLDDMD

SEQ ID NO: 36022 - protein, 9 aa, synthetic construct
GGSGLDEIF

SEQ ID NO: 36023 - protein, 9 aa, synthetic construct
GGSGLDELN

SEQ ID NO: 36024 - protein, 9 aa, synthetic construct
GGSGLDFLE

SEQ ID NO: 36025 - protein, 9 aa, synthetic construct
GGSGLDFLQ

SEQ ID NO: 36026 - protein, 9 aa, synthetic construct
GGSGLDGLL

SEQ ID NO: 36027 - protein, 9 aa, synthetic construct
GGSGLDHFR

SEQ ID NO: 36028 - protein, 9 aa, synthetic construct
GGSGLDHLI

SEQ ID NO: 36029 - protein, 9 aa, synthetic construct
GGSGLDHLN

SEQ ID NO: 36030 - protein, 9 aa, synthetic construct
GGSGLDIFR

SEQ ID NO: 36031 - protein, 9 aa, synthetic construct
GGSGLDIIN

SEQ ID NO: 36032 - protein, 9 aa, synthetic construct
GGSGLDIIV

SEQ ID NO: 36033 - protein, 9 aa, synthetic construct
GGSGKDTII

SEQ ID NO: 36034 - protein, 9 aa, synthetic construct
GGSGKDTID

SEQ ID NO: 36035 - protein, 9 aa, synthetic construct
GGSGKDLIK

SEQ ID NO: 36036 - protein, 9 aa, synthetic construct
GGSGKDQVL

SEQ ID NO: 36037 - protein, 9 aa, synthetic construct
GGSGKDLLG

SEQ ID NO: 36038 - protein, 9 aa, synthetic construct
GGSGKDLLT

SEQ ID NO: 36039 - protein, 9 aa, synthetic construct
GGSGKDLMT

SEQ ID NO: 36040 - protein, 9 aa, synthetic construct
GGSGKDMLI

SEQ ID NO: 36041 - protein, 9 aa, synthetic construct
GGSGKDMLS

SEQ ID NO: 36042 - protein, 9 aa, synthetic construct
GGSGKDMLV

SEQ ID NO: 36043 - protein, 9 aa, synthetic construct
GGSGKDNIS

SEQ ID NO: 36044 - protein, 9 aa, synthetic construct
GGSGKDNIW

SEQ ID NO: 36045 - protein, 9 aa, synthetic construct
GGSGKDNLY

SEQ ID NO: 36046 - protein, 9 aa, synthetic construct
GGSGKDQIE

SEQ ID NO: 36047 - protein, 9 aa, synthetic construct
GGSGKDQIK

SEQ ID NO: 36048 - protein, 9 aa, synthetic construct
GGSGKDQIQ

SEQ ID NO: 36049 - protein, 9 aa, synthetic construct
GGSGKDQLI

SEQ ID NO: 36050 - protein, 9 aa, synthetic construct
GGSGKDRIA

SEQ ID NO: 36051 - protein, 9 aa, synthetic construct
GGSGKDTFT

SEQ ID NO: 36052 - protein, 9 aa, synthetic construct
GGSGKDRIF

SEQ ID NO: 36053 - protein, 9 aa, synthetic construct
GGSGKDRIY

SEQ ID NO: 36054 - protein, 9 aa, synthetic construct
GGSGKDRVK

SEQ ID NO: 36055 - protein, 9 aa, synthetic construct
GGSGKDRVQ

SEQ ID NO: 36056 - protein, 9 aa, synthetic construct
GGSGKDSFI

SEQ ID NO: 36057 - protein, 9 aa, synthetic construct
GGSGKDSIF

SEQ ID NO: 36058 - protein, 9 aa, synthetic construct
GGSGKDSLL

SEQ ID NO: 36059 - protein, 9 aa, synthetic construct
GGSGKDSLQ

SEQ ID NO: 36060 - protein, 9 aa, synthetic construct
GGSGKDSVN

SEQ ID NO: 36061 - protein, 9 aa, synthetic construct
GGSGKDSVS

SEQ ID NO: 36062 - protein, 9 aa, synthetic construct
GGSGKDTAT

SEQ ID NO: 36063 - protein, 9 aa, synthetic construct
GGSGKDTFI

SEQ ID NO: 36064 - protein, 9 aa, synthetic construct
GGSGKDTFL

SEQ ID NO: 36065 - protein, 9 aa, synthetic construct
GGSGIDSLI

SEQ ID NO: 36066 - protein, 9 aa, synthetic construct
GGSGIDSAS

SEQ ID NO: 36067 - protein, 9 aa, synthetic construct
GGSGHDILS

SEQ ID NO: 36068 - protein, 9 aa, synthetic construct
GGSGIDRML

SEQ ID NO: 36069 - protein, 9 aa, synthetic construct
GGSGHDRIL

SEQ ID NO: 36070 - protein, 9 aa, synthetic construct
GGSGHDRIY

SEQ ID NO: 36071 - protein, 9 aa, synthetic construct
GGSGHDRLD

SEQ ID NO: 36072 - protein, 9 aa, synthetic construct
GGSGHDRLG

SEQ ID NO: 36073 - protein, 9 aa, synthetic construct
GGSGHDRLV

SEQ ID NO: 36074 - protein, 9 aa, synthetic construct
GGSGHDRME

SEQ ID NO: 36075 - protein, 9 aa, synthetic construct
GGSGHDRMI

SEQ ID NO: 36076 - protein, 9 aa, synthetic construct
GGSGHDRVE

SEQ ID NO: 36077 - protein, 9 aa, synthetic construct
GGSGHDRYF

SEQ ID NO: 36078 - protein, 9 aa, synthetic construct
GGSGHDRYL

SEQ ID NO: 36079 - protein, 9 aa, synthetic construct
GGSGHDSIE

SEQ ID NO: 36080 - protein, 9 aa, synthetic construct
GGSGHDSLE

SEQ ID NO: 36081 - protein, 9 aa, synthetic construct
GGSGHDSLS

SEQ ID NO: 36082 - protein, 9 aa, synthetic construct
GGSGHDSLV

SEQ ID NO: 36083 - protein, 9 aa, synthetic construct
GGSGHDSMS

SEQ ID NO: 36084 - protein, 9 aa, synthetic construct
GGSGHDSMY

SEQ ID NO: 36085 - protein, 9 aa, synthetic construct
GGSGHDTAI

SEQ ID NO: 36086 - protein, 9 aa, synthetic construct
GGSGHDTAM

SEQ ID NO: 36087 - protein, 9 aa, synthetic construct
GGSGHDTFY

SEQ ID NO: 36088 - protein, 9 aa, synthetic construct
GGSGHDTIA

SEQ ID NO: 36089 - protein, 9 aa, synthetic construct
GGSGHDTID

SEQ ID NO: 36090 - protein, 9 aa, synthetic construct
GGSGHDTIF

SEQ ID NO: 36091 - protein, 9 aa, synthetic construct
GGSGHDTIN

SEQ ID NO: 36092 - protein, 9 aa, synthetic construct
GGSGHDTIR

SEQ ID NO: 36093 - protein, 9 aa, synthetic construct
GGSGHDTIW

SEQ ID NO: 36094 - protein, 9 aa, synthetic construct
GGSGHDTLF

SEQ ID NO: 36095 - protein, 9 aa, synthetic construct
GGSGHDTLV

SEQ ID NO: 36096 - protein, 9 aa, synthetic construct
GGSGHDTMR

SEQ ID NO: 36097 - protein, 9 aa, synthetic construct
GGSGHDTMS

SEQ ID NO: 36098 - protein, 9 aa, synthetic construct
GGSGHDRIF

SEQ ID NO: 36099 - protein, 9 aa, synthetic construct
GGSGHDRIE

SEQ ID NO: 36100 - protein, 9 aa, synthetic construct
GGSGHDRFV

SEQ ID NO: 36101 - protein, 9 aa, synthetic construct
GGSGHDLVN

SEQ ID NO: 36102 - protein, 9 aa, synthetic construct
GGSGHDKID

SEQ ID NO: 36103 - protein, 9 aa, synthetic construct
GGSGHDKIL

SEQ ID NO: 36104 - protein, 9 aa, synthetic construct
GGSGHDKLE

SEQ ID NO: 36105 - protein, 9 aa, synthetic construct
GGSGHDKLN

SEQ ID NO: 36106 - protein, 9 aa, synthetic construct
GGSGHDLFG

SEQ ID NO: 36107 - protein, 9 aa, synthetic construct
GGSGHDLIQ

SEQ ID NO: 36108 - protein, 9 aa, synthetic construct
GGSGHDLIR

SEQ ID NO: 36109 - protein, 9 aa, synthetic construct
GGSGHDLLA

SEQ ID NO: 36110 - protein, 9 aa, synthetic construct
GGSGHDLLD

SEQ ID NO: 36111 - protein, 9 aa, synthetic construct
GGSGHDLLE

SEQ ID NO: 36112 - protein, 9 aa, synthetic construct
GGSGHDLLI

SEQ ID NO: 36113 - protein, 9 aa, synthetic construct
GGSGHDLLV

SEQ ID NO: 36114 - protein, 9 aa, synthetic construct
GGSGHDLMD

SEQ ID NO: 36115 - protein, 9 aa, synthetic construct
GGSGHDMID

SEQ ID NO: 36116 - protein, 9 aa, synthetic construct
GGSGHDQMF

SEQ ID NO: 36117 - protein, 9 aa, synthetic construct
GGSGHDMIL

SEQ ID NO: 36118 - protein, 9 aa, synthetic construct
GGSGHDMIN

SEQ ID NO: 36119 - protein, 9 aa, synthetic construct
GGSGHDMLD

SEQ ID NO: 36120 - protein, 9 aa, synthetic construct
GGSGHDNLN

SEQ ID NO: 36121 - protein, 9 aa, synthetic construct
GGSGHDNLQ

SEQ ID NO: 36122 - protein, 9 aa, synthetic construct
GGSGHDNLT

SEQ ID NO: 36123 - protein, 9 aa, synthetic construct
GGSGHDNMT

SEQ ID NO: 36124 - protein, 9 aa, synthetic construct
GGSGHDQIV

SEQ ID NO: 36125 - protein, 9 aa, synthetic construct
GGSGHDQLD

SEQ ID NO: 36126 - protein, 9 aa, synthetic construct
GGSGHDQLE

SEQ ID NO: 36127 - protein, 9 aa, synthetic construct
GGSGHDQLF

SEQ ID NO: 36128 - protein, 9 aa, synthetic construct
GGSGHDQLH

SEQ ID NO: 36129 - protein, 9 aa, synthetic construct
GGSGHDQLS

SEQ ID NO: 36130 - protein, 9 aa, synthetic construct
GGSGHDTVF

SEQ ID NO: 36131 - protein, 9 aa, synthetic construct
GGSGHDTYV

SEQ ID NO: 36132 - protein, 9 aa, synthetic construct
GGSGHDVFR

SEQ ID NO: 36133 - protein, 9 aa, synthetic construct
GGSGIDLMV

SEQ ID NO: 36134 - protein, 9 aa, synthetic construct
GGSGIDIFA

SEQ ID NO: 36135 - protein, 9 aa, synthetic construct
GGSGIDIFV

SEQ ID NO: 36136 - protein, 9 aa, synthetic construct
GGSGIDIIF

SEQ ID NO: 36137 - protein, 9 aa, synthetic construct
GGSGIDILL

SEQ ID NO: 36138 - protein, 9 aa, synthetic construct
GGSGIDILT

SEQ ID NO: 36139 - protein, 9 aa, synthetic construct
GGSGIDIMT

SEQ ID NO: 36140 - protein, 9 aa, synthetic construct
GGSGIDIVF

SEQ ID NO: 36141 - protein, 9 aa, synthetic construct
GGSGIDKLR

SEQ ID NO: 36142 - protein, 9 aa, synthetic construct
GGSGIDLIW

SEQ ID NO: 36143 - protein, 9 aa, synthetic construct
GGSGIDLLN

SEQ ID NO: 36144 - protein, 9 aa, synthetic construct
GGSGIDLLQ

SEQ ID NO: 36145 - protein, 9 aa, synthetic construct
GGSGIDLLV

SEQ ID NO: 36146 - protein, 9 aa, synthetic construct
GGSGIDLML

SEQ ID NO: 36147 - protein, 9 aa, synthetic construct
GGSGIDLVW

SEQ ID NO: 36148 - protein, 9 aa, synthetic construct
GGSGIDGVI

SEQ ID NO: 36149 - protein, 9 aa, synthetic construct
GGSGIDMAS

SEQ ID NO: 36150 - protein, 9 aa, synthetic construct
GGSGIDNLV

SEQ ID NO: 36151 - protein, 9 aa, synthetic construct
GGSGIDQFV

SEQ ID NO: 36152 - protein, 9 aa, synthetic construct
GGSGIDQID

SEQ ID NO: 36153 - protein, 9 aa, synthetic construct
GGSGIDQME

SEQ ID NO: 36154 - protein, 9 aa, synthetic construct
GGSGIDQML

SEQ ID NO: 36155 - protein, 9 aa, synthetic construct
GGSGIDRAI

SEQ ID NO: 36156 - protein, 9 aa, synthetic construct
GGSGIDRIF

SEQ ID NO: 36157 - protein, 9 aa, synthetic construct
GGSGIDRLF

SEQ ID NO: 36158 - protein, 9 aa, synthetic construct
GGSGIDRLI

SEQ ID NO: 36159 - protein, 9 aa, synthetic construct
GGSGIDRLN

SEQ ID NO: 36160 - protein, 9 aa, synthetic construct
GGSGIDRLT

SEQ ID NO: 36161 - protein, 9 aa, synthetic construct
GGSGIDRLY

SEQ ID NO: 36162 - protein, 9 aa, synthetic construct
GGSGIDHAS

SEQ ID NO: 36163 - protein, 9 aa, synthetic construct
GGSGIDFMA

SEQ ID NO: 36164 - protein, 9 aa, synthetic construct
GGSGHDVID

SEQ ID NO: 36165 - protein, 9 aa, synthetic construct
GGSGHDWLW

SEQ ID NO: 36166 - protein, 9 aa, synthetic construct
GGSGHDVIG

SEQ ID NO: 36167 - protein, 9 aa, synthetic construct
GGSGHDVIL

SEQ ID NO: 36168 - protein, 9 aa, synthetic construct
GGSGHDVIT

SEQ ID NO: 36169 - protein, 9 aa, synthetic construct
GGSGHDVLE

SEQ ID NO: 36170 - protein, 9 aa, synthetic construct
GGSGHDVLF

SEQ ID NO: 36171 - protein, 9 aa, synthetic construct
GGSGHDVLH

SEQ ID NO: 36172 - protein, 9 aa, synthetic construct
GGSGHDVLQ

SEQ ID NO: 36173 - protein, 9 aa, synthetic construct
GGSGHDVLS

SEQ ID NO: 36174 - protein, 9 aa, synthetic construct
GGSGHDVMA

SEQ ID NO: 36175 - protein, 9 aa, synthetic construct
GGSGHDVMI

SEQ ID NO: 36176 - protein, 9 aa, synthetic construct
GGSGHDVMR

SEQ ID NO: 36177 - protein, 9 aa, synthetic construct
GGSGHDWLA

SEQ ID NO: 36178 - protein, 9 aa, synthetic construct
GGSGHDWLR

SEQ ID NO: 36179 - protein, 9 aa, synthetic construct
GGSGHDWVY

SEQ ID NO: 36180 - protein, 9 aa, synthetic construct
GGSGIDFLV

SEQ ID NO: 36181 - protein, 9 aa, synthetic construct
GGSGHDYID

SEQ ID NO: 36182 - protein, 9 aa, synthetic construct
GGSGHDYLF

SEQ ID NO: 36183 - protein, 9 aa, synthetic construct
GGSGHDYLM

SEQ ID NO: 36184 - protein, 9 aa, synthetic construct
GGSGHDYLN

SEQ ID NO: 36185 - protein, 9 aa, synthetic construct
GGSGIDAAS

SEQ ID NO: 36186 - protein, 9 aa, synthetic construct
GGSGIDAFS

SEQ ID NO: 36187 - protein, 9 aa, synthetic construct
GGSGIDALH

SEQ ID NO: 36188 - protein, 9 aa, synthetic construct
GGSGIDALN

SEQ ID NO: 36189 - protein, 9 aa, synthetic construct
GGSGIDAVV

SEQ ID NO: 36190 - protein, 9 aa, synthetic construct
GGSGIDAYH

SEQ ID NO: 36191 - protein, 9 aa, synthetic construct
GGSGIDFAM

SEQ ID NO: 36192 - protein, 9 aa, synthetic construct
GGSGIDFIT

SEQ ID NO: 36193 - protein, 9 aa, synthetic construct
GGSGIDFLF

SEQ ID NO: 36194 - protein, 9 aa, synthetic construct
GGRGNDAFD

SEQ ID NO: 36195 - protein, 9 aa, synthetic construct
GGRGMDVMF

SEQ ID NO: 36196 - protein, 9 aa, synthetic construct
GGRGMDTLR

SEQ ID NO: 36197 - protein, 9 aa, synthetic construct
GGQGADTFT

SEQ ID NO: 36198 - protein, 9 aa, synthetic construct
GGQGADRIS

SEQ ID NO: 36199 - protein, 9 aa, synthetic construct
GGQGADRLD

SEQ ID NO: 36200 - protein, 9 aa, synthetic construct
GGQGADRLG

SEQ ID NO: 36201 - protein, 9 aa, synthetic construct
GGQGADRLM

SEQ ID NO: 36202 - protein, 9 aa, synthetic construct
GGQGADRLR

SEQ ID NO: 36203 - protein, 9 aa, synthetic construct
GGQGADRLW

SEQ ID NO: 36204 - protein, 9 aa, synthetic construct
GGQGADRMA

SEQ ID NO: 36205 - protein, 9 aa, synthetic construct
GGQGADSID

SEQ ID NO: 36206 - protein, 9 aa, synthetic construct
GGQGADSIG

SEQ ID NO: 36207 - protein, 9 aa, synthetic construct
GGQGADSIL

SEQ ID NO: 36208 - protein, 9 aa, synthetic construct
GGQGADSIN

SEQ ID NO: 36209 - protein, 9 aa, synthetic construct
GGQGADSIQ

SEQ ID NO: 36210 - protein, 9 aa, synthetic construct
GGQGADSIR

SEQ ID NO: 36211 - protein, 9 aa, synthetic construct
GGQGADSIS

SEQ ID NO: 36212 - protein, 9 aa, synthetic construct
GGQGADSIT

SEQ ID NO: 36213 - protein, 9 aa, synthetic construct
GGQGADSLD

SEQ ID NO: 36214 - protein, 9 aa, synthetic construct
GGQGADSLG

SEQ ID NO: 36215 - protein, 9 aa, synthetic construct
GGQGADSLI

SEQ ID NO: 36216 - protein, 9 aa, synthetic construct
GGQGADSLL

SEQ ID NO: 36217 - protein, 9 aa, synthetic construct
GGQGADSLM

SEQ ID NO: 36218 - protein, 9 aa, synthetic construct
GGQGADSLN

SEQ ID NO: 36219 - protein, 9 aa, synthetic construct
GGQGADSLV

SEQ ID NO: 36220 - protein, 9 aa, synthetic construct
GGQGADSME

SEQ ID NO: 36221 - protein, 9 aa, synthetic construct
GGQGADSMF

SEQ ID NO: 36222 - protein, 9 aa, synthetic construct
GGQGADSMV

SEQ ID NO: 36223 - protein, 9 aa, synthetic construct
GGQGADSVD

SEQ ID NO: 36224 - protein, 9 aa, synthetic construct
GGQGADSVN

SEQ ID NO: 36225 - protein, 9 aa, synthetic construct
GGQGADTAV

SEQ ID NO: 36226 - protein, 9 aa, synthetic construct
GGQGADTFA

SEQ ID NO: 36227 - protein, 9 aa, synthetic construct
GGQGADRIA

SEQ ID NO: 36228 - protein, 9 aa, synthetic construct
GGQGADQVF

SEQ ID NO: 36229 - protein, 9 aa, synthetic construct
GGQGADQLR

SEQ ID NO: 36230 - protein, 9 aa, synthetic construct
GGQGADLFI

SEQ ID NO: 36231 - protein, 9 aa, synthetic construct
GGQGADHID

SEQ ID NO: 36232 - protein, 9 aa, synthetic construct
GGQGADHLF

SEQ ID NO: 36233 - protein, 9 aa, synthetic construct
GGQGADHLH

SEQ ID NO: 36234 - protein, 9 aa, synthetic construct
GGQGADHLI

SEQ ID NO: 36235 - protein, 9 aa, synthetic construct
GGQGADHLL

SEQ ID NO: 36236 - protein, 9 aa, synthetic construct
GGQGADIFI

SEQ ID NO: 36237 - protein, 9 aa, synthetic construct
GGQGADIFR

SEQ ID NO: 36238 - protein, 9 aa, synthetic construct
GGQGADILA

SEQ ID NO: 36239 - protein, 9 aa, synthetic construct
GGQGADILS

SEQ ID NO: 36240 - protein, 9 aa, synthetic construct
GGQGADKFC

SEQ ID NO: 36241 - protein, 9 aa, synthetic construct
GGQGADKID

SEQ ID NO: 36242 - protein, 9 aa, synthetic construct
GGQGADKLL

SEQ ID NO: 36243 - protein, 9 aa, synthetic construct
GGQGADKLW

SEQ ID NO: 36244 - protein, 9 aa, synthetic construct
GGQGADLIE

SEQ ID NO: 36245 - protein, 9 aa, synthetic construct
GGQGADQLF

SEQ ID NO: 36246 - protein, 9 aa, synthetic construct
GGQGADLLL

SEQ ID NO: 36247 - protein, 9 aa, synthetic construct
GGQGADLLQ

SEQ ID NO: 36248 - protein, 9 aa, synthetic construct
GGQGADLLY

SEQ ID NO: 36249 - protein, 9 aa, synthetic construct
GGQGADLMD

SEQ ID NO: 36250 - protein, 9 aa, synthetic construct
GGQGADLMY

SEQ ID NO: 36251 - protein, 9 aa, synthetic construct
GGQGADMLF

SEQ ID NO: 36252 - protein, 9 aa, synthetic construct
GGQGADNIA

SEQ ID NO: 36253 - protein, 9 aa, synthetic construct
GGQGADNLN

SEQ ID NO: 36254 - protein, 9 aa, synthetic construct
GGQGADNLS

SEQ ID NO: 36255 - protein, 9 aa, synthetic construct
GGQGADNMT

SEQ ID NO: 36256 - protein, 9 aa, synthetic construct
GGQGADQFF

SEQ ID NO: 36257 - protein, 9 aa, synthetic construct
GGQGADQFV

SEQ ID NO: 36258 - protein, 9 aa, synthetic construct
GGQGADQIL

SEQ ID NO: 36259 - protein, 9 aa, synthetic construct
GGQGADTFE

SEQ ID NO: 36260 - protein, 9 aa, synthetic construct
GGQGADTIF

SEQ ID NO: 36261 - protein, 9 aa, synthetic construct
GGQGDDFVH

SEQ ID NO: 36262 - protein, 9 aa, synthetic construct
GGQGADTIR

SEQ ID NO: 36263 - protein, 9 aa, synthetic construct
GGQGADYVY

SEQ ID NO: 36264 - protein, 9 aa, synthetic construct
GGQGCDTLK

SEQ ID NO: 36265 - protein, 9 aa, synthetic construct
GGQGCDTYV

SEQ ID NO: 36266 - protein, 9 aa, synthetic construct
GGQGDDAIL

SEQ ID NO: 36267 - protein, 9 aa, synthetic construct
GGQGDDAIS

SEQ ID NO: 36268 - protein, 9 aa, synthetic construct
GGQGDDALT

SEQ ID NO: 36269 - protein, 9 aa, synthetic construct
GGQGDDAVE

SEQ ID NO: 36270 - protein, 9 aa, synthetic construct
GGQGDDCID

SEQ ID NO: 36271 - protein, 9 aa, synthetic construct
GGQGDDDIL

SEQ ID NO: 36272 - protein, 9 aa, synthetic construct
GGQGDDDIR

SEQ ID NO: 36273 - protein, 9 aa, synthetic construct
GGQGDDDIS

SEQ ID NO: 36274 - protein, 9 aa, synthetic construct
GGQGDDDIV

SEQ ID NO: 36275 - protein, 9 aa, synthetic construct
GGQGDDDLF

SEQ ID NO: 36276 - protein, 9 aa, synthetic construct
GGQGDDDML

SEQ ID NO: 36277 - protein, 9 aa, synthetic construct
GGQGDDDVR

SEQ ID NO: 36278 - protein, 9 aa, synthetic construct
GGQGDDELA

SEQ ID NO: 36279 - protein, 9 aa, synthetic construct
GGQGDDELN

SEQ ID NO: 36280 - protein, 9 aa, synthetic construct
GGQGDDELS

SEQ ID NO: 36281 - protein, 9 aa, synthetic construct
GGQGDDELY

SEQ ID NO: 36282 - protein, 9 aa, synthetic construct
GGQGDDEVR

SEQ ID NO: 36283 - protein, 9 aa, synthetic construct
GGQGDDEVS

SEQ ID NO: 36284 - protein, 9 aa, synthetic construct
GGQGDDEVY

SEQ ID NO: 36285 - protein, 9 aa, synthetic construct
GGQGDDFAQ

SEQ ID NO: 36286 - protein, 9 aa, synthetic construct
GGQGDDFII

SEQ ID NO: 36287 - protein, 9 aa, synthetic construct
GGQGDDFIM

SEQ ID NO: 36288 - protein, 9 aa, synthetic construct
GGQGDDFIN

SEQ ID NO: 36289 - protein, 9 aa, synthetic construct
GGQGDDFLE

SEQ ID NO: 36290 - protein, 9 aa, synthetic construct
GGQGDDFLI

SEQ ID NO: 36291 - protein, 9 aa, synthetic construct
GGQGDDFLL

SEQ ID NO: 36292 - protein, 9 aa, synthetic construct
GGQGADYVS

SEQ ID NO: 36293 - protein, 9 aa, synthetic construct
GGQGADYLY

SEQ ID NO: 36294 - protein, 9 aa, synthetic construct
GGQGADWMD

SEQ ID NO: 36295 - protein, 9 aa, synthetic construct
GGQGADTVY

SEQ ID NO: 36296 - protein, 9 aa, synthetic construct
GGQGADTIY

SEQ ID NO: 36297 - protein, 9 aa, synthetic construct
GGQGADTMD

SEQ ID NO: 36298 - protein, 9 aa, synthetic construct
GGQGADTML

SEQ ID NO: 36299 - protein, 9 aa, synthetic construct
GGQGADTMN

SEQ ID NO: 36300 - protein, 9 aa, synthetic construct
GGQGADTMV

SEQ ID NO: 36301 - protein, 9 aa, synthetic construct
GGQGADTVA

SEQ ID NO: 36302 - protein, 9 aa, synthetic construct
GGQGADTVD

SEQ ID NO: 36303 - protein, 9 aa, synthetic construct
GGQGADTVF

SEQ ID NO: 36304 - protein, 9 aa, synthetic construct
GGQGADTVH

SEQ ID NO: 36305 - protein, 9 aa, synthetic construct
GGQGADTVK

SEQ ID NO: 36306 - protein, 9 aa, synthetic construct
GGQGADTVL

SEQ ID NO: 36307 - protein, 9 aa, synthetic construct
GGQGADTVN

SEQ ID NO: 36308 - protein, 9 aa, synthetic construct
GGQGADTVR

SEQ ID NO: 36309 - protein, 9 aa, synthetic construct
GGQGADVAV

SEQ ID NO: 36310 - protein, 9 aa, synthetic construct
GGQGADWLN

SEQ ID NO: 36311 - protein, 9 aa, synthetic construct
GGQGADVFR

SEQ ID NO: 36312 - protein, 9 aa, synthetic construct
GGQGADVIF

SEQ ID NO: 36313 - protein, 9 aa, synthetic construct
GGQGADVIK

SEQ ID NO: 36314 - protein, 9 aa, synthetic construct
GGQGADVIN

SEQ ID NO: 36315 - protein, 9 aa, synthetic construct
GGQGADVLE

SEQ ID NO: 36316 - protein, 9 aa, synthetic construct
GGQGADVLF

SEQ ID NO: 36317 - protein, 9 aa, synthetic construct
GGQGADVLY

SEQ ID NO: 36318 - protein, 9 aa, synthetic construct
GGQGADVMH

SEQ ID NO: 36319 - protein, 9 aa, synthetic construct
GGQGADVMI

SEQ ID NO: 36320 - protein, 9 aa, synthetic construct
GGQGADVMM

SEQ ID NO: 36321 - protein, 9 aa, synthetic construct
GGQGADVYV

SEQ ID NO: 36322 - protein, 9 aa, synthetic construct
GGQGADWIH

SEQ ID NO: 36323 - protein, 9 aa, synthetic construct
GGQGADWLE

SEQ ID NO: 36324 - protein, 9 aa, synthetic construct
GGQGADGLK

SEQ ID NO: 36325 - protein, 9 aa, synthetic construct
GGQGADFVQ

SEQ ID NO: 36326 - protein, 9 aa, synthetic construct
GGQGADFLD

SEQ ID NO: 36327 - protein, 9 aa, synthetic construct
GGQGADFIQ

SEQ ID NO: 36328 - protein, 9 aa, synthetic construct
GGPGSDWID

SEQ ID NO: 36329 - protein, 9 aa, synthetic construct
GGPGSDWLL

SEQ ID NO: 36330 - protein, 9 aa, synthetic construct
GGPGSDWLY

SEQ ID NO: 36331 - protein, 9 aa, synthetic construct
GGPGSDWVL

SEQ ID NO: 36332 - protein, 9 aa, synthetic construct
GGPGSDYIA

SEQ ID NO: 36333 - protein, 9 aa, synthetic construct
GGPGSDYIE

SEQ ID NO: 36334 - protein, 9 aa, synthetic construct
GGPGSDYIQ

SEQ ID NO: 36335 - protein, 9 aa, synthetic construct
GGPGTDAFM

SEQ ID NO: 36336 - protein, 9 aa, synthetic construct
GGPGTDAVY

SEQ ID NO: 36337 - protein, 9 aa, synthetic construct
GGPGTDFFE

SEQ ID NO: 36338 - protein, 9 aa, synthetic construct
GGPGTDFIA

SEQ ID NO: 36339 - protein, 9 aa, synthetic construct
GGPGTDFLF

SEQ ID NO: 36340 - protein, 9 aa, synthetic construct
GGPGTDHLY

SEQ ID NO: 36341 - protein, 9 aa, synthetic construct
GGPGTDHMF

SEQ ID NO: 36342 - protein, 9 aa, synthetic construct
GGPGTDIAV

SEQ ID NO: 36343 - protein, 9 aa, synthetic construct
GGPGTDIFV

SEQ ID NO: 36344 - protein, 9 aa, synthetic construct
GGPGTDILI

SEQ ID NO: 36345 - protein, 9 aa, synthetic construct
GGPGTDILS

SEQ ID NO: 36346 - protein, 9 aa, synthetic construct
GGPGTDILY

SEQ ID NO: 36347 - protein, 9 aa, synthetic construct
GGPGTDIMN

SEQ ID NO: 36348 - protein, 9 aa, synthetic construct
GGPGTDLID

SEQ ID NO: 36349 - protein, 9 aa, synthetic construct
GGPGTDLLT

SEQ ID NO: 36350 - protein, 9 aa, synthetic construct
GGPGTDLLY

SEQ ID NO: 36351 - protein, 9 aa, synthetic construct
GGPGTDLVD

SEQ ID NO: 36352 - protein, 9 aa, synthetic construct
GGPGTDNFD

SEQ ID NO: 36353 - protein, 9 aa, synthetic construct
GGPGTDQLF

SEQ ID NO: 36354 - protein, 9 aa, synthetic construct
GGPGTDQLT

SEQ ID NO: 36355 - protein, 9 aa, synthetic construct
GGPGTDQLY

SEQ ID NO: 36356 - protein, 9 aa, synthetic construct
GGPGTDRLN

SEQ ID NO: 36357 - protein, 9 aa, synthetic construct
GGPGSDWAV

SEQ ID NO: 36358 - protein, 9 aa, synthetic construct
GGPGSDVYI

SEQ ID NO: 36359 - protein, 9 aa, synthetic construct
GGPGSDVMI

SEQ ID NO: 36360 - protein, 9 aa, synthetic construct
GGPGSDTFK

SEQ ID NO: 36361 - protein, 9 aa, synthetic construct
GGPGSDQLN

SEQ ID NO: 36362 - protein, 9 aa, synthetic construct
GGPGSDRFF

SEQ ID NO: 36363 - protein, 9 aa, synthetic construct
GGPGSDRIS

SEQ ID NO: 36364 - protein, 9 aa, synthetic construct
GGPGSDRIY

SEQ ID NO: 36365 - protein, 9 aa, synthetic construct
GGPGSDRLF

SEQ ID NO: 36366 - protein, 9 aa, synthetic construct
GGPGSDRLG

SEQ ID NO: 36367 - protein, 9 aa, synthetic construct
GGPGSDRMT

SEQ ID NO: 36368 - protein, 9 aa, synthetic construct
GGPGSDRMV

SEQ ID NO: 36369 - protein, 9 aa, synthetic construct
GGPGSDSIS

SEQ ID NO: 36370 - protein, 9 aa, synthetic construct
GGPGSDSLL

SEQ ID NO: 36371 - protein, 9 aa, synthetic construct
GGPGSDSLN

SEQ ID NO: 36372 - protein, 9 aa, synthetic construct
GGPGSDTAG

SEQ ID NO: 36373 - protein, 9 aa, synthetic construct
GGPGSDTAV

SEQ ID NO: 36374 - protein, 9 aa, synthetic construct
GGPGSDTIF

SEQ ID NO: 36375 - protein, 9 aa, synthetic construct
GGPGSDVLT

SEQ ID NO: 36376 - protein, 9 aa, synthetic construct
GGPGSDTLA

SEQ ID NO: 36377 - protein, 9 aa, synthetic construct
GGPGSDTLN

SEQ ID NO: 36378 - protein, 9 aa, synthetic construct
GGPGSDTMS

SEQ ID NO: 36379 - protein, 9 aa, synthetic construct
GGPGSDTVD

SEQ ID NO: 36380 - protein, 9 aa, synthetic construct
GGPGSDTVI

SEQ ID NO: 36381 - protein, 9 aa, synthetic construct
GGPGSDTVR

SEQ ID NO: 36382 - protein, 9 aa, synthetic construct
GGPGSDTVS

SEQ ID NO: 36383 - protein, 9 aa, synthetic construct
GGPGSDTYH

SEQ ID NO: 36384 - protein, 9 aa, synthetic construct
GGPGSDVAF

SEQ ID NO: 36385 - protein, 9 aa, synthetic construct
GGPGSDVIN

SEQ ID NO: 36386 - protein, 9 aa, synthetic construct
GGPGSDVLD

SEQ ID NO: 36387 - protein, 9 aa, synthetic construct
GGPGSDVLF

SEQ ID NO: 36388 - protein, 9 aa, synthetic construct
GGPGSDVLH

SEQ ID NO: 36389 - protein, 9 aa, synthetic construct
GGPGTDRLQ

SEQ ID NO: 36390 - protein, 9 aa, synthetic construct
GGPGTDSLW

SEQ ID NO: 36391 - protein, 9 aa, synthetic construct
GGPGTDTAD

SEQ ID NO: 36392 - protein, 9 aa, synthetic construct
GGQGADALY

SEQ ID NO: 36393 - protein, 9 aa, synthetic construct
GGPGYDELY

SEQ ID NO: 36394 - protein, 9 aa, synthetic construct
GGPGYDIAS

SEQ ID NO: 36395 - protein, 9 aa, synthetic construct
GGPGYDLLF

SEQ ID NO: 36396 - protein, 9 aa, synthetic construct
GGPGYDLMI

SEQ ID NO: 36397 - protein, 9 aa, synthetic construct
GGPGYDLMT

SEQ ID NO: 36398 - protein, 9 aa, synthetic construct
GGPGYDNLT

SEQ ID NO: 36399 - protein, 9 aa, synthetic construct
GGPGYDRLW

SEQ ID NO: 36400 - protein, 9 aa, synthetic construct
GGPGYDSLW

SEQ ID NO: 36401 - protein, 9 aa, synthetic construct
GGPGYDTLF

SEQ ID NO: 36402 - protein, 9 aa, synthetic construct
GGPGYDVLI

SEQ ID NO: 36403 - protein, 9 aa, synthetic construct
GGQGADAAD

SEQ ID NO: 36404 - protein, 9 aa, synthetic construct
GGQGADAFI

SEQ ID NO: 36405 - protein, 9 aa, synthetic construct
GGQGADALH

SEQ ID NO: 36406 - protein, 9 aa, synthetic construct
GGQGADAMI

SEQ ID NO: 36407 - protein, 9 aa, synthetic construct
GGPGWDQLR

SEQ ID NO: 36408 - protein, 9 aa, synthetic construct
GGQGADDLD

SEQ ID NO: 36409 - protein, 9 aa, synthetic construct
GGQGADDLF

SEQ ID NO: 36410 - protein, 9 aa, synthetic construct
GGQGADDLW

SEQ ID NO: 36411 - protein, 9 aa, synthetic construct
GGQGADDLY

SEQ ID NO: 36412 - protein, 9 aa, synthetic construct
GGQGADDYY

SEQ ID NO: 36413 - protein, 9 aa, synthetic construct
GGQGADEFR

SEQ ID NO: 36414 - protein, 9 aa, synthetic construct
GGQGADEIN

SEQ ID NO: 36415 - protein, 9 aa, synthetic construct
GGQGADEIY

SEQ ID NO: 36416 - protein, 9 aa, synthetic construct
GGQGADELS

SEQ ID NO: 36417 - protein, 9 aa, synthetic construct
GGQGADELV

SEQ ID NO: 36418 - protein, 9 aa, synthetic construct
GGQGADELW

SEQ ID NO: 36419 - protein, 9 aa, synthetic construct
GGQGADELY

SEQ ID NO: 36420 - protein, 9 aa, synthetic construct
GGQGADEVS

SEQ ID NO: 36421 - protein, 9 aa, synthetic construct
GGPGXDTLL

SEQ ID NO: 36422 - protein, 9 aa, synthetic construct
GGPGWDELY

SEQ ID NO: 36423 - protein, 9 aa, synthetic construct
GGPGTDTFA

SEQ ID NO: 36424 - protein, 9 aa, synthetic construct
GGPGVDFLF

SEQ ID NO: 36425 - protein, 9 aa, synthetic construct
GGPGTDTLD

SEQ ID NO: 36426 - protein, 9 aa, synthetic construct
GGPGTDTLE

SEQ ID NO: 36427 - protein, 9 aa, synthetic construct
GGPGTDTLI

SEQ ID NO: 36428 - protein, 9 aa, synthetic construct
GGPGTDTLL

SEQ ID NO: 36429 - protein, 9 aa, synthetic construct
GGPGTDTLV

SEQ ID NO: 36430 - protein, 9 aa, synthetic construct
GGPGTDTVL

SEQ ID NO: 36431 - protein, 9 aa, synthetic construct
GGPGTDVLR

SEQ ID NO: 36432 - protein, 9 aa, synthetic construct
GGPGTDVLV

SEQ ID NO: 36433 - protein, 9 aa, synthetic construct
GGPGTDWLK

SEQ ID NO: 36434 - protein, 9 aa, synthetic construct
GGPGTDWLM

SEQ ID NO: 36435 - protein, 9 aa, synthetic construct
GGPGTDYLV

SEQ ID NO: 36436 - protein, 9 aa, synthetic construct
GGPGVDAMS

SEQ ID NO: 36437 - protein, 9 aa, synthetic construct
GGPGVDELY

SEQ ID NO: 36438 - protein, 9 aa, synthetic construct
GGPGVDFVR

SEQ ID NO: 36439 - protein, 9 aa, synthetic construct
GGPGVDVLD

SEQ ID NO: 36440 - protein, 9 aa, synthetic construct
GGPGVDKLY

SEQ ID NO: 36441 - protein, 9 aa, synthetic construct
GGPGVDRLV

SEQ ID NO: 36442 - protein, 9 aa, synthetic construct
GGPGVDRME

SEQ ID NO: 36443 - protein, 9 aa, synthetic construct
GGPGVDRMV

SEQ ID NO: 36444 - protein, 9 aa, synthetic construct
GGPGVDSAH

SEQ ID NO: 36445 - protein, 9 aa, synthetic construct
GGPGVDSAY

SEQ ID NO: 36446 - protein, 9 aa, synthetic construct
GGPGVDSIR

SEQ ID NO: 36447 - protein, 9 aa, synthetic construct
GGPGVDSLQ

SEQ ID NO: 36448 - protein, 9 aa, synthetic construct
GGPGVDTLL

SEQ ID NO: 36449 - protein, 9 aa, synthetic construct
GGPGVDTLN

SEQ ID NO: 36450 - protein, 9 aa, synthetic construct
GGPGVDTLR

SEQ ID NO: 36451 - protein, 9 aa, synthetic construct
GGPGVDTLT

SEQ ID NO: 36452 - protein, 9 aa, synthetic construct
GGPGVDTVD

SEQ ID NO: 36453 - protein, 9 aa, synthetic construct
GGQGDDFLN

SEQ ID NO: 36454 - protein, 9 aa, synthetic construct
GGQGDDFVQ

SEQ ID NO: 36455 - protein, 9 aa, synthetic construct
GGQGHDYLE

SEQ ID NO: 36456 - protein, 9 aa, synthetic construct
GGQGGDLIL

SEQ ID NO: 36457 - protein, 9 aa, synthetic construct
GGQGEDTLK

SEQ ID NO: 36458 - protein, 9 aa, synthetic construct
GGQGEDTMA

SEQ ID NO: 36459 - protein, 9 aa, synthetic construct
GGQGEDVIF

SEQ ID NO: 36460 - protein, 9 aa, synthetic construct
GGQGEDVLE

SEQ ID NO: 36461 - protein, 9 aa, synthetic construct
GGQGEDVLQ

SEQ ID NO: 36462 - protein, 9 aa, synthetic construct
GGQGEDVMF

SEQ ID NO: 36463 - protein, 9 aa, synthetic construct
GGQGEDWLD

SEQ ID NO: 36464 - protein, 9 aa, synthetic construct
GGQGEDWLE

SEQ ID NO: 36465 - protein, 9 aa, synthetic construct
GGQGEDYLD

SEQ ID NO: 36466 - protein, 9 aa, synthetic construct
GGQGEDYLV

SEQ ID NO: 36467 - protein, 9 aa, synthetic construct
GGQGFDALY

SEQ ID NO: 36468 - protein, 9 aa, synthetic construct
GGQGFDCLS

SEQ ID NO: 36469 - protein, 9 aa, synthetic construct
GGQGFDFAR

SEQ ID NO: 36470 - protein, 9 aa, synthetic construct
GGQGFDHLF

SEQ ID NO: 36471 - protein, 9 aa, synthetic construct
GGQGFDIMS

SEQ ID NO: 36472 - protein, 9 aa, synthetic construct
GGQGFDRFL

SEQ ID NO: 36473 - protein, 9 aa, synthetic construct
GGQGFDRIA

SEQ ID NO: 36474 - protein, 9 aa, synthetic construct
GGQGFDRLF

SEQ ID NO: 36475 - protein, 9 aa, synthetic construct
GGQGFDTIQ

SEQ ID NO: 36476 - protein, 9 aa, synthetic construct
GGQGFDYAI

SEQ ID NO: 36477 - protein, 9 aa, synthetic construct
GGQGFDYLF

SEQ ID NO: 36478 - protein, 9 aa, synthetic construct
GGQGGDEIR

SEQ ID NO: 36479 - protein, 9 aa, synthetic construct
GGQGGDELI

SEQ ID NO: 36480 - protein, 9 aa, synthetic construct
GGQGGDFID

SEQ ID NO: 36481 - protein, 9 aa, synthetic construct
GGQGGDHII

SEQ ID NO: 36482 - protein, 9 aa, synthetic construct
GGQGGDHLE

SEQ ID NO: 36483 - protein, 9 aa, synthetic construct
GGQGGDILF

SEQ ID NO: 36484 - protein, 9 aa, synthetic construct
GGQGGDILH

SEQ ID NO: 36485 - protein, 9 aa, synthetic construct
GGQGGDILT

SEQ ID NO: 36486 - protein, 9 aa, synthetic construct
GGQGEDTLE

SEQ ID NO: 36487 - protein, 9 aa, synthetic construct
GGQGEDTIN

SEQ ID NO: 36488 - protein, 9 aa, synthetic construct
GGQGEDTID

SEQ ID NO: 36489 - protein, 9 aa, synthetic construct
GGQGEDFLN

SEQ ID NO: 36490 - protein, 9 aa, synthetic construct
GGQGDDVYY

SEQ ID NO: 36491 - protein, 9 aa, synthetic construct
GGQGDDWID

SEQ ID NO: 36492 - protein, 9 aa, synthetic construct
GGQGDDWLD

SEQ ID NO: 36493 - protein, 9 aa, synthetic construct
GGQGDDWLG

SEQ ID NO: 36494 - protein, 9 aa, synthetic construct
GGQGDDWMH

SEQ ID NO: 36495 - protein, 9 aa, synthetic construct
GGQGDDWVD

SEQ ID NO: 36496 - protein, 9 aa, synthetic construct
GGQGDDWVV

SEQ ID NO: 36497 - protein, 9 aa, synthetic construct
GGQGDDYLA

SEQ ID NO: 36498 - protein, 9 aa, synthetic construct
GGQGDDYLI

SEQ ID NO: 36499 - protein, 9 aa, synthetic construct
GGQGEDALY

SEQ ID NO: 36500 - protein, 9 aa, synthetic construct
GGQGEDDID

SEQ ID NO: 36501 - protein, 9 aa, synthetic construct
GGQGEDELH

SEQ ID NO: 36502 - protein, 9 aa, synthetic construct
GGQGEDELY

SEQ ID NO: 36503 - protein, 9 aa, synthetic construct
GGQGEDHFQ

SEQ ID NO: 36504 - protein, 9 aa, synthetic construct
GGQGEDSLE

SEQ ID NO: 36505 - protein, 9 aa, synthetic construct
GGQGEDIFK

SEQ ID NO: 36506 - protein, 9 aa, synthetic construct
GGQGEDILQ

SEQ ID NO: 36507 - protein, 9 aa, synthetic construct
GGQGEDILY

SEQ ID NO: 36508 - protein, 9 aa, synthetic construct
GGQGEDIVD

SEQ ID NO: 36509 - protein, 9 aa, synthetic construct
GGQGEDKFM

SEQ ID NO: 36510 - protein, 9 aa, synthetic construct
GGQGEDLLD

SEQ ID NO: 36511 - protein, 9 aa, synthetic construct
GGQGEDLVF

SEQ ID NO: 36512 - protein, 9 aa, synthetic construct
GGQGEDLVY

SEQ ID NO: 36513 - protein, 9 aa, synthetic construct
GGQGEDQLR

SEQ ID NO: 36514 - protein, 9 aa, synthetic construct
GGQGEDRIL

SEQ ID NO: 36515 - protein, 9 aa, synthetic construct
GGQGEDRLH

SEQ ID NO: 36516 - protein, 9 aa, synthetic construct
GGQGEDRLL

SEQ ID NO: 36517 - protein, 9 aa, synthetic construct
GGQGEDSIF

SEQ ID NO: 36518 - protein, 9 aa, synthetic construct
GGQGGDILY

SEQ ID NO: 36519 - protein, 9 aa, synthetic construct
GGQGGDLLN

SEQ ID NO: 36520 - protein, 9 aa, synthetic construct
GGQGDDGLD

SEQ ID NO: 36521 - protein, 9 aa, synthetic construct
GGQGGDLLV

SEQ ID NO: 36522 - protein, 9 aa, synthetic construct
GGQGHDFID

SEQ ID NO: 36523 - protein, 9 aa, synthetic construct
GGQGHDFLM

SEQ ID NO: 36524 - protein, 9 aa, synthetic construct
GGQGHDFLR

SEQ ID NO: 36525 - protein, 9 aa, synthetic construct
GGQGHDHLW

SEQ ID NO: 36526 - protein, 9 aa, synthetic construct
GGQGHDILI

SEQ ID NO: 36527 - protein, 9 aa, synthetic construct
GGQGHDILL

SEQ ID NO: 36528 - protein, 9 aa, synthetic construct
GGQGHDILW

SEQ ID NO: 36529 - protein, 9 aa, synthetic construct
GGQGHDKMR

SEQ ID NO: 36530 - protein, 9 aa, synthetic construct
GGQGHDLIG

SEQ ID NO: 36531 - protein, 9 aa, synthetic construct
GGQGHDLIY

SEQ ID NO: 36532 - protein, 9 aa, synthetic construct
GGQGHDLLT

SEQ ID NO: 36533 - protein, 9 aa, synthetic construct
GGQGHDLMI

SEQ ID NO: 36534 - protein, 9 aa, synthetic construct
GGQGHDMLS

SEQ ID NO: 36535 - protein, 9 aa, synthetic construct
GGQGHDQIW

SEQ ID NO: 36536 - protein, 9 aa, synthetic construct
GGQGHDQLH

SEQ ID NO: 36537 - protein, 9 aa, synthetic construct
GGQGHDRLA

SEQ ID NO: 36538 - protein, 9 aa, synthetic construct
GGQGHDRLD

SEQ ID NO: 36539 - protein, 9 aa, synthetic construct
GGQGHDRLE

SEQ ID NO: 36540 - protein, 9 aa, synthetic construct
GGQGHDRLL

SEQ ID NO: 36541 - protein, 9 aa, synthetic construct
GGQGHDRLR

SEQ ID NO: 36542 - protein, 9 aa, synthetic construct
GGQGHDRLW

SEQ ID NO: 36543 - protein, 9 aa, synthetic construct
GGQGHDSLR

SEQ ID NO: 36544 - protein, 9 aa, synthetic construct
GGQGHDSLT

SEQ ID NO: 36545 - protein, 9 aa, synthetic construct
GGQGHDTLA

SEQ ID NO: 36546 - protein, 9 aa, synthetic construct
GGQGHDTLS

SEQ ID NO: 36547 - protein, 9 aa, synthetic construct
GGQGHDTLV

SEQ ID NO: 36548 - protein, 9 aa, synthetic construct
GGQGHDTLY

SEQ ID NO: 36549 - protein, 9 aa, synthetic construct
GGQGHDVIL

SEQ ID NO: 36550 - protein, 9 aa, synthetic construct
GGQGHDVLS

SEQ ID NO: 36551 - protein, 9 aa, synthetic construct
GGQGHDELD

SEQ ID NO: 36552 - protein, 9 aa, synthetic construct
GGQGHDEIY

SEQ ID NO: 36553 - protein, 9 aa, synthetic construct
GGQGHDDME

SEQ ID NO: 36554 - protein, 9 aa, synthetic construct
GGQGGDTLI

SEQ ID NO: 36555 - protein, 9 aa, synthetic construct
GGQGGDLVL

SEQ ID NO: 36556 - protein, 9 aa, synthetic construct
GGQGGDNLS

SEQ ID NO: 36557 - protein, 9 aa, synthetic construct
GGQGGDQIF

SEQ ID NO: 36558 - protein, 9 aa, synthetic construct
GGQGGDRIE

SEQ ID NO: 36559 - protein, 9 aa, synthetic construct
GGQGGDRLE

SEQ ID NO: 36560 - protein, 9 aa, synthetic construct
GGQGGDRLY

SEQ ID NO: 36561 - protein, 9 aa, synthetic construct
GGQGGDSII

SEQ ID NO: 36562 - protein, 9 aa, synthetic construct
GGQGGDSIL

SEQ ID NO: 36563 - protein, 9 aa, synthetic construct
GGQGGDSIV

SEQ ID NO: 36564 - protein, 9 aa, synthetic construct
GGQGGDSLI

SEQ ID NO: 36565 - protein, 9 aa, synthetic construct
GGQGGDSMT

SEQ ID NO: 36566 - protein, 9 aa, synthetic construct
GGQGGDTFS

SEQ ID NO: 36567 - protein, 9 aa, synthetic construct
GGQGGDTLG

SEQ ID NO: 36568 - protein, 9 aa, synthetic construct
GGQGGDTLL

SEQ ID NO: 36569 - protein, 9 aa, synthetic construct
GGQGHDALY

SEQ ID NO: 36570 - protein, 9 aa, synthetic construct
GGQGGDTLS

SEQ ID NO: 36571 - protein, 9 aa, synthetic construct
GGQGGDTLV

SEQ ID NO: 36572 - protein, 9 aa, synthetic construct
GGQGGDTVF

SEQ ID NO: 36573 - protein, 9 aa, synthetic construct
GGQGGDTVH

SEQ ID NO: 36574 - protein, 9 aa, synthetic construct
GGQGGDTYL

SEQ ID NO: 36575 - protein, 9 aa, synthetic construct
GGQGGDVFV

SEQ ID NO: 36576 - protein, 9 aa, synthetic construct
GGQGGDVIY

SEQ ID NO: 36577 - protein, 9 aa, synthetic construct
GGQGGDVLL

SEQ ID NO: 36578 - protein, 9 aa, synthetic construct
GGQGGDWAE

SEQ ID NO: 36579 - protein, 9 aa, synthetic construct
GGQGGDWLE

SEQ ID NO: 36580 - protein, 9 aa, synthetic construct
GGQGGDWML

SEQ ID NO: 36581 - protein, 9 aa, synthetic construct
GGQGGDYLD

SEQ ID NO: 36582 - protein, 9 aa, synthetic construct
GGQGGDYLY

SEQ ID NO: 36583 - protein, 9 aa, synthetic construct
GGQGDDVYI

SEQ ID NO: 36584 - protein, 9 aa, synthetic construct
GGQGDDVVY

SEQ ID NO: 36585 - protein, 9 aa, synthetic construct
GGQGDDVVE

SEQ ID NO: 36586 - protein, 9 aa, synthetic construct
GGQGDDVVD

SEQ ID NO: 36587 - protein, 9 aa, synthetic construct
GGQGDDLAI

SEQ ID NO: 36588 - protein, 9 aa, synthetic construct
GGQGDDLFL

SEQ ID NO: 36589 - protein, 9 aa, synthetic construct
GGQGDDLFQ

SEQ ID NO: 36590 - protein, 9 aa, synthetic construct
GGQGDDLIA

SEQ ID NO: 36591 - protein, 9 aa, synthetic construct
GGQGDDLIF

SEQ ID NO: 36592 - protein, 9 aa, synthetic construct
GGQGDDLIH

SEQ ID NO: 36593 - protein, 9 aa, synthetic construct
GGQGDDLIN

SEQ ID NO: 36594 - protein, 9 aa, synthetic construct
GGQGDDLIS

SEQ ID NO: 36595 - protein, 9 aa, synthetic construct
GGQGDDLIV

SEQ ID NO: 36596 - protein, 9 aa, synthetic construct
GGQGDDLLC

SEQ ID NO: 36597 - protein, 9 aa, synthetic construct
GGQGDDLLM

SEQ ID NO: 36598 - protein, 9 aa, synthetic construct
GGQGDDLLY

SEQ ID NO: 36599 - protein, 9 aa, synthetic construct
GGQGDDLMT

SEQ ID NO: 36600 - protein, 9 aa, synthetic construct
GGQGDDLVD

SEQ ID NO: 36601 - protein, 9 aa, synthetic construct
GGQGDDLVL

SEQ ID NO: 36602 - protein, 9 aa, synthetic construct
GGQGDDLVN

SEQ ID NO: 36603 - protein, 9 aa, synthetic construct
GGQGDDLVQ

SEQ ID NO: 36604 - protein, 9 aa, synthetic construct
GGQGDDLVR

SEQ ID NO: 36605 - protein, 9 aa, synthetic construct
GGQGDDLYL

SEQ ID NO: 36606 - protein, 9 aa, synthetic construct
GGQGDDMAI

SEQ ID NO: 36607 - protein, 9 aa, synthetic construct
GGQGDDMLR

SEQ ID NO: 36608 - protein, 9 aa, synthetic construct
GGQGDDMMD

SEQ ID NO: 36609 - protein, 9 aa, synthetic construct
GGQGDDMVF

SEQ ID NO: 36610 - protein, 9 aa, synthetic construct
GGQGDDMVS

SEQ ID NO: 36611 - protein, 9 aa, synthetic construct
GGQGDDNFI

SEQ ID NO: 36612 - protein, 9 aa, synthetic construct
GGQGDDNIA

SEQ ID NO: 36613 - protein, 9 aa, synthetic construct
GGQGDDNIT

SEQ ID NO: 36614 - protein, 9 aa, synthetic construct
GGQGDDNLI

SEQ ID NO: 36615 - protein, 9 aa, synthetic construct
GGQGDDNLN

SEQ ID NO: 36616 - protein, 9 aa, synthetic construct
GGQGDDKMW

SEQ ID NO: 36617 - protein, 9 aa, synthetic construct
GGQGDDKLY

SEQ ID NO: 36618 - protein, 9 aa, synthetic construct
GGQGDDKLW

SEQ ID NO: 36619 - protein, 9 aa, synthetic construct
GGQGDDIAL

SEQ ID NO: 36620 - protein, 9 aa, synthetic construct
GGQGDDGLI

SEQ ID NO: 36621 - protein, 9 aa, synthetic construct
GGQGDDGLS

SEQ ID NO: 36622 - protein, 9 aa, synthetic construct
GGQGDDGLT

SEQ ID NO: 36623 - protein, 9 aa, synthetic construct
GGQGDDGYT

SEQ ID NO: 36624 - protein, 9 aa, synthetic construct
GGQGDDHIN

SEQ ID NO: 36625 - protein, 9 aa, synthetic construct
GGQGDDHIQ

SEQ ID NO: 36626 - protein, 9 aa, synthetic construct
GGQGDDHIS

SEQ ID NO: 36627 - protein, 9 aa, synthetic construct
GGQGDDHLD

SEQ ID NO: 36628 - protein, 9 aa, synthetic construct
GGQGDDHLE

SEQ ID NO: 36629 - protein, 9 aa, synthetic construct
GGQGDDHLN

SEQ ID NO: 36630 - protein, 9 aa, synthetic construct
GGQGDDHLV

SEQ ID NO: 36631 - protein, 9 aa, synthetic construct
GGQGDDHMR

SEQ ID NO: 36632 - protein, 9 aa, synthetic construct
GGQGDDHVS

SEQ ID NO: 36633 - protein, 9 aa, synthetic construct
GGQGDDIIE

SEQ ID NO: 36634 - protein, 9 aa, synthetic construct
GGQGDDKLF

SEQ ID NO: 36635 - protein, 9 aa, synthetic construct
GGQGDDIIM

SEQ ID NO: 36636 - protein, 9 aa, synthetic construct
GGQGDDIIN

SEQ ID NO: 36637 - protein, 9 aa, synthetic construct
GGQGDDIIY

SEQ ID NO: 36638 - protein, 9 aa, synthetic construct
GGQGDDILA

SEQ ID NO: 36639 - protein, 9 aa, synthetic construct
GGQGDDIVI

SEQ ID NO: 36640 - protein, 9 aa, synthetic construct
GGQGDDIVL

SEQ ID NO: 36641 - protein, 9 aa, synthetic construct
GGQGDDIVN

SEQ ID NO: 36642 - protein, 9 aa, synthetic construct
GGQGDDIVQ

SEQ ID NO: 36643 - protein, 9 aa, synthetic construct
GGQGDDIVT

SEQ ID NO: 36644 - protein, 9 aa, synthetic construct
GGQGDDKID

SEQ ID NO: 36645 - protein, 9 aa, synthetic construct
GGQGDDKIF

SEQ ID NO: 36646 - protein, 9 aa, synthetic construct
GGQGDDKIL

SEQ ID NO: 36647 - protein, 9 aa, synthetic construct
GGQGDDKLE

SEQ ID NO: 36648 - protein, 9 aa, synthetic construct
GGQGDDNLS

SEQ ID NO: 36649 - protein, 9 aa, synthetic construct
GGQGDDNLV

SEQ ID NO: 36650 - protein, 9 aa, synthetic construct
GGQGDDNLY

SEQ ID NO: 36651 - protein, 9 aa, synthetic construct
GGQGDDTVN

SEQ ID NO: 36652 - protein, 9 aa, synthetic construct
GGQGDDSYL

SEQ ID NO: 36653 - protein, 9 aa, synthetic construct
GGQGDDTAF

SEQ ID NO: 36654 - protein, 9 aa, synthetic construct
GGQGDDTAI

SEQ ID NO: 36655 - protein, 9 aa, synthetic construct
GGQGDDTFM

SEQ ID NO: 36656 - protein, 9 aa, synthetic construct
GGQGDDTFV

SEQ ID NO: 36657 - protein, 9 aa, synthetic construct
GGQGDDTFY

SEQ ID NO: 36658 - protein, 9 aa, synthetic construct
GGQGDDTIQ

SEQ ID NO: 36659 - protein, 9 aa, synthetic construct
GGQGDDTIW

SEQ ID NO: 36660 - protein, 9 aa, synthetic construct
GGQGDDTMA

SEQ ID NO: 36661 - protein, 9 aa, synthetic construct
GGQGDDTMD

SEQ ID NO: 36662 - protein, 9 aa, synthetic construct
GGQGDDTVH

SEQ ID NO: 36663 - protein, 9 aa, synthetic construct
GGQGDDTVI

SEQ ID NO: 36664 - protein, 9 aa, synthetic construct
GGQGDDTVM

SEQ ID NO: 36665 - protein, 9 aa, synthetic construct
GGQGDDTVR

SEQ ID NO: 36666 - protein, 9 aa, synthetic construct
GGQGDDSVS

SEQ ID NO: 36667 - protein, 9 aa, synthetic construct
GGQGDDTYF

SEQ ID NO: 36668 - protein, 9 aa, synthetic construct
GGQGDDTYR

SEQ ID NO: 36669 - protein, 9 aa, synthetic construct
GGQGDDVAY

SEQ ID NO: 36670 - protein, 9 aa, synthetic construct
GGQGDDVFD

SEQ ID NO: 36671 - protein, 9 aa, synthetic construct
GGQGDDVFV

SEQ ID NO: 36672 - protein, 9 aa, synthetic construct
GGQGDDVIG

SEQ ID NO: 36673 - protein, 9 aa, synthetic construct
GGQGDDVIK

SEQ ID NO: 36674 - protein, 9 aa, synthetic construct
GGQGDDVIN

SEQ ID NO: 36675 - protein, 9 aa, synthetic construct
GGQGDDVLK

SEQ ID NO: 36676 - protein, 9 aa, synthetic construct
GGQGDDVLW

SEQ ID NO: 36677 - protein, 9 aa, synthetic construct
GGQGDDVMA

SEQ ID NO: 36678 - protein, 9 aa, synthetic construct
GGQGDDVMD

SEQ ID NO: 36679 - protein, 9 aa, synthetic construct
GGQGDDVMT

SEQ ID NO: 36680 - protein, 9 aa, synthetic construct
GGQGDDSVV

SEQ ID NO: 36681 - protein, 9 aa, synthetic construct
GGQGDDSVL

SEQ ID NO: 36682 - protein, 9 aa, synthetic construct
GGQGDDQID

SEQ ID NO: 36683 - protein, 9 aa, synthetic construct
GGQGDDRLT

SEQ ID NO: 36684 - protein, 9 aa, synthetic construct
GGQGDDQLE

SEQ ID NO: 36685 - protein, 9 aa, synthetic construct
GGQGDDQLL

SEQ ID NO: 36686 - protein, 9 aa, synthetic construct
GGQGDDQLQ

SEQ ID NO: 36687 - protein, 9 aa, synthetic construct
GGQGDDQMF

SEQ ID NO: 36688 - protein, 9 aa, synthetic construct
GGQGDDQMQ

SEQ ID NO: 36689 - protein, 9 aa, synthetic construct
GGQGDDQVV

SEQ ID NO: 36690 - protein, 9 aa, synthetic construct
GGQGDDQVY

SEQ ID NO: 36691 - protein, 9 aa, synthetic construct
GGQGDDRAY

SEQ ID NO: 36692 - protein, 9 aa, synthetic construct
GGQGDDRFI

SEQ ID NO: 36693 - protein, 9 aa, synthetic construct
GGQGDDRID

SEQ ID NO: 36694 - protein, 9 aa, synthetic construct
GGQGDDRIT

SEQ ID NO: 36695 - protein, 9 aa, synthetic construct
GGQGDDRIV

SEQ ID NO: 36696 - protein, 9 aa, synthetic construct
GGQGDDRLM

SEQ ID NO: 36697 - protein, 9 aa, synthetic construct
GGQGDDRVD

SEQ ID NO: 36698 - protein, 9 aa, synthetic construct
GGQGDDSVE

SEQ ID NO: 36699 - protein, 9 aa, synthetic construct
GGQGDDRVE

SEQ ID NO: 36700 - protein, 9 aa, synthetic construct
GGQGDDRYM

SEQ ID NO: 36701 - protein, 9 aa, synthetic construct
GGQGDDSFL

SEQ ID NO: 36702 - protein, 9 aa, synthetic construct
GGQGDDSIA

SEQ ID NO: 36703 - protein, 9 aa, synthetic construct
GGQGDDSIE

SEQ ID NO: 36704 - protein, 9 aa, synthetic construct
GGQGDDSIF

SEQ ID NO: 36705 - protein, 9 aa, synthetic construct
GGQGDDSIH

SEQ ID NO: 36706 - protein, 9 aa, synthetic construct
GGQGDDSIK

SEQ ID NO: 36707 - protein, 9 aa, synthetic construct
GGQGDDSIT

SEQ ID NO: 36708 - protein, 9 aa, synthetic construct
GGQGDDSIV

SEQ ID NO: 36709 - protein, 9 aa, synthetic construct
GGQGDDSLE

SEQ ID NO: 36710 - protein, 9 aa, synthetic construct
GGQGDDSME

SEQ ID NO: 36711 - protein, 9 aa, synthetic construct
GGQGDDSMT

SEQ ID NO: 36712 - protein, 9 aa, synthetic construct
GGPGSDQLL

SEQ ID NO: 36713 - protein, 9 aa, synthetic construct
GGPGSDQLA

SEQ ID NO: 36714 - protein, 9 aa, synthetic construct
GGPGSDMLL

SEQ ID NO: 36715 - protein, 9 aa, synthetic construct
GGPGKDTIA

SEQ ID NO: 36716 - protein, 9 aa, synthetic construct
GGPGIDIMD

SEQ ID NO: 36717 - protein, 9 aa, synthetic construct
GGPGIDKIY

SEQ ID NO: 36718 - protein, 9 aa, synthetic construct
GGPGIDLIE

SEQ ID NO: 36719 - protein, 9 aa, synthetic construct
GGPGIDLLF

SEQ ID NO: 36720 - protein, 9 aa, synthetic construct
GGPGIDLVW

SEQ ID NO: 36721 - protein, 9 aa, synthetic construct
GGPGIDNLR

SEQ ID NO: 36722 - protein, 9 aa, synthetic construct
GGPGIDRAH

SEQ ID NO: 36723 - protein, 9 aa, synthetic construct
GGPGIDRLV

SEQ ID NO: 36724 - protein, 9 aa, synthetic construct
GGPGIDSMS

SEQ ID NO: 36725 - protein, 9 aa, synthetic construct
GGPGIDTAI

SEQ ID NO: 36726 - protein, 9 aa, synthetic construct
GGPGIDTLS

SEQ ID NO: 36727 - protein, 9 aa, synthetic construct
GGPGIDTLT

SEQ ID NO: 36728 - protein, 9 aa, synthetic construct
GGPGIDTLW

SEQ ID NO: 36729 - protein, 9 aa, synthetic construct
GGPGIDTVD

SEQ ID NO: 36730 - protein, 9 aa, synthetic construct
GGPGIDTVG

SEQ ID NO: 36731 - protein, 9 aa, synthetic construct
GGPGIDTYR

SEQ ID NO: 36732 - protein, 9 aa, synthetic construct
GGPGIDVMI

SEQ ID NO: 36733 - protein, 9 aa, synthetic construct
GGPGIDVVD

SEQ ID NO: 36734 - protein, 9 aa, synthetic construct
GGPGKDAFV

SEQ ID NO: 36735 - protein, 9 aa, synthetic construct
GGPGKDFLF

SEQ ID NO: 36736 - protein, 9 aa, synthetic construct
GGPGKDKLK

SEQ ID NO: 36737 - protein, 9 aa, synthetic construct
GGPGKDLIT

SEQ ID NO: 36738 - protein, 9 aa, synthetic construct
GGPGKDLLT

SEQ ID NO: 36739 - protein, 9 aa, synthetic construct
GGPGKDNIF

SEQ ID NO: 36740 - protein, 9 aa, synthetic construct
GGPGKDQLA

SEQ ID NO: 36741 - protein, 9 aa, synthetic construct
GGPGKDRLI

SEQ ID NO: 36742 - protein, 9 aa, synthetic construct
GGPGKDSFV

SEQ ID NO: 36743 - protein, 9 aa, synthetic construct
GGPGKDSLT

SEQ ID NO: 36744 - protein, 9 aa, synthetic construct
GGPGKDSLV

SEQ ID NO: 36745 - protein, 9 aa, synthetic construct
GGPGIDILS

SEQ ID NO: 36746 - protein, 9 aa, synthetic construct
GGPGIDILD

SEQ ID NO: 36747 - protein, 9 aa, synthetic construct
GGPGIDFLA

SEQ ID NO: 36748 - protein, 9 aa, synthetic construct
GGPGHDTLT

SEQ ID NO: 36749 - protein, 9 aa, synthetic construct
GGPGHDLMY

SEQ ID NO: 36750 - protein, 9 aa, synthetic construct
GGPGHDNIN

SEQ ID NO: 36751 - protein, 9 aa, synthetic construct
GGPGHDNLD

SEQ ID NO: 36752 - protein, 9 aa, synthetic construct
GGPGHDQLD

SEQ ID NO: 36753 - protein, 9 aa, synthetic construct
GGPGHDQMR

SEQ ID NO: 36754 - protein, 9 aa, synthetic construct
GGPGHDRLE

SEQ ID NO: 36755 - protein, 9 aa, synthetic construct
GGPGHDRLF

SEQ ID NO: 36756 - protein, 9 aa, synthetic construct
GGPGHDRLL

SEQ ID NO: 36757 - protein, 9 aa, synthetic construct
GGPGHDRLY

SEQ ID NO: 36758 - protein, 9 aa, synthetic construct
GGPGHDRMT

SEQ ID NO: 36759 - protein, 9 aa, synthetic construct
GGPGHDTIH

SEQ ID NO: 36760 - protein, 9 aa, synthetic construct
GGPGHDTLA

SEQ ID NO: 36761 - protein, 9 aa, synthetic construct
GGPGHDTLN

SEQ ID NO: 36762 - protein, 9 aa, synthetic construct
GGPGHDTLV

SEQ ID NO: 36763 - protein, 9 aa, synthetic construct
GGPGIDAVD

SEQ ID NO: 36764 - protein, 9 aa, synthetic construct
GGPGHDTYF

SEQ ID NO: 36765 - protein, 9 aa, synthetic construct
GGPGHDTYI

SEQ ID NO: 36766 - protein, 9 aa, synthetic construct
GGPGHDVAN

SEQ ID NO: 36767 - protein, 9 aa, synthetic construct
GGPGHDVID

SEQ ID NO: 36768 - protein, 9 aa, synthetic construct
GGPGHDVIH

SEQ ID NO: 36769 - protein, 9 aa, synthetic construct
GGPGHDVIY

SEQ ID NO: 36770 - protein, 9 aa, synthetic construct
GGPGHDVLD

SEQ ID NO: 36771 - protein, 9 aa, synthetic construct
GGPGHDVLE

SEQ ID NO: 36772 - protein, 9 aa, synthetic construct
GGPGHDVLL

SEQ ID NO: 36773 - protein, 9 aa, synthetic construct
GGPGHDVVA

SEQ ID NO: 36774 - protein, 9 aa, synthetic construct
GGPGHDWIV

SEQ ID NO: 36775 - protein, 9 aa, synthetic construct
GGPGIDAAG

SEQ ID NO: 36776 - protein, 9 aa, synthetic construct
GGPGIDALY

SEQ ID NO: 36777 - protein, 9 aa, synthetic construct
GGPGKDSML

SEQ ID NO: 36778 - protein, 9 aa, synthetic construct
GGPGKDTLL

SEQ ID NO: 36779 - protein, 9 aa, synthetic construct
GGPGSDMIY

SEQ ID NO: 36780 - protein, 9 aa, synthetic construct
GGPGKDTLS

SEQ ID NO: 36781 - protein, 9 aa, synthetic construct
GGPGNDAIR

SEQ ID NO: 36782 - protein, 9 aa, synthetic construct
GGPGNDALE

SEQ ID NO: 36783 - protein, 9 aa, synthetic construct
GGPGNDALT

SEQ ID NO: 36784 - protein, 9 aa, synthetic construct
GGPGNDAVY

SEQ ID NO: 36785 - protein, 9 aa, synthetic construct
GGPGNDAYF

SEQ ID NO: 36786 - protein, 9 aa, synthetic construct
GGPGNDDID

SEQ ID NO: 36787 - protein, 9 aa, synthetic construct
GGPGNDDIE

SEQ ID NO: 36788 - protein, 9 aa, synthetic construct
GGPGNDDIQ

SEQ ID NO: 36789 - protein, 9 aa, synthetic construct
GGPGNDDIR

SEQ ID NO: 36790 - protein, 9 aa, synthetic construct
GGPGNDDLD

SEQ ID NO: 36791 - protein, 9 aa, synthetic construct
GGPGNDDLF

SEQ ID NO: 36792 - protein, 9 aa, synthetic construct
GGPGNDEIR

SEQ ID NO: 36793 - protein, 9 aa, synthetic construct
GGPGNDEIY

SEQ ID NO: 36794 - protein, 9 aa, synthetic construct
GGPGNDELD

SEQ ID NO: 36795 - protein, 9 aa, synthetic construct
GGPGNDELL

SEQ ID NO: 36796 - protein, 9 aa, synthetic construct
GGPGNDELN

SEQ ID NO: 36797 - protein, 9 aa, synthetic construct
GGPGNDELV

SEQ ID NO: 36798 - protein, 9 aa, synthetic construct
GGPGNDEMD

SEQ ID NO: 36799 - protein, 9 aa, synthetic construct
GGPGNDEVH

SEQ ID NO: 36800 - protein, 9 aa, synthetic construct
GGPGNDFIG

SEQ ID NO: 36801 - protein, 9 aa, synthetic construct
GGPGNDFIH

SEQ ID NO: 36802 - protein, 9 aa, synthetic construct
GGPGNDFIT

SEQ ID NO: 36803 - protein, 9 aa, synthetic construct
GGPGNDFLF

SEQ ID NO: 36804 - protein, 9 aa, synthetic construct
GGPGNDFLT

SEQ ID NO: 36805 - protein, 9 aa, synthetic construct
GGPGNDFMN

SEQ ID NO: 36806 - protein, 9 aa, synthetic construct
GGPGNDGLL

SEQ ID NO: 36807 - protein, 9 aa, synthetic construct
GGPGNDGLT

SEQ ID NO: 36808 - protein, 9 aa, synthetic construct
GGPGNDGLW

SEQ ID NO: 36809 - protein, 9 aa, synthetic construct
GGPGNDHIF

SEQ ID NO: 36810 - protein, 9 aa, synthetic construct
GGPGNDAIN

SEQ ID NO: 36811 - protein, 9 aa, synthetic construct
GGPGNDAIK

SEQ ID NO: 36812 - protein, 9 aa, synthetic construct
GGPGMDRLL

SEQ ID NO: 36813 - protein, 9 aa, synthetic construct
GGPGLDALH

SEQ ID NO: 36814 - protein, 9 aa, synthetic construct
GGPGKDTLV

SEQ ID NO: 36815 - protein, 9 aa, synthetic construct
GGPGKDTVS

SEQ ID NO: 36816 - protein, 9 aa, synthetic construct
GGPGKDVAF

SEQ ID NO: 36817 - protein, 9 aa, synthetic construct
GGPGKDVFL

SEQ ID NO: 36818 - protein, 9 aa, synthetic construct
GGPGKDVFR

SEQ ID NO: 36819 - protein, 9 aa, synthetic construct
GGPGKDVIN

SEQ ID NO: 36820 - protein, 9 aa, synthetic construct
GGPGKDVIS

SEQ ID NO: 36821 - protein, 9 aa, synthetic construct
GGPGKDVIV

SEQ ID NO: 36822 - protein, 9 aa, synthetic construct
GGPGKDVLN

SEQ ID NO: 36823 - protein, 9 aa, synthetic construct
GGPGKDVLS

SEQ ID NO: 36824 - protein, 9 aa, synthetic construct
GGPGKDVLV

SEQ ID NO: 36825 - protein, 9 aa, synthetic construct
GGPGKDVLY

SEQ ID NO: 36826 - protein, 9 aa, synthetic construct
GGPGKDWMS

SEQ ID NO: 36827 - protein, 9 aa, synthetic construct
GGPGLDLAI

SEQ ID NO: 36828 - protein, 9 aa, synthetic construct
GGPGMDRLD

SEQ ID NO: 36829 - protein, 9 aa, synthetic construct
GGPGLDLLL

SEQ ID NO: 36830 - protein, 9 aa, synthetic construct
GGPGLDLLW

SEQ ID NO: 36831 - protein, 9 aa, synthetic construct
GGPGLDMLD

SEQ ID NO: 36832 - protein, 9 aa, synthetic construct
GGPGLDQLS

SEQ ID NO: 36833 - protein, 9 aa, synthetic construct
GGPGLDRAI

SEQ ID NO: 36834 - protein, 9 aa, synthetic construct
GGPGLDRLF

SEQ ID NO: 36835 - protein, 9 aa, synthetic construct
GGPGLDRLT

SEQ ID NO: 36836 - protein, 9 aa, synthetic construct
GGPGLDSLD

SEQ ID NO: 36837 - protein, 9 aa, synthetic construct
GGPGLDTIV

SEQ ID NO: 36838 - protein, 9 aa, synthetic construct
GGPGLDVYV

SEQ ID NO: 36839 - protein, 9 aa, synthetic construct
GGPGLDYLV

SEQ ID NO: 36840 - protein, 9 aa, synthetic construct
GGPGMDHLH

SEQ ID NO: 36841 - protein, 9 aa, synthetic construct
GGPGMDMAH

SEQ ID NO: 36842 - protein, 9 aa, synthetic construct
GGPGHDLMF

SEQ ID NO: 36843 - protein, 9 aa, synthetic construct
GGPGHDLLV

SEQ ID NO: 36844 - protein, 9 aa, synthetic construct
GGPGHDLLF

SEQ ID NO: 36845 - protein, 9 aa, synthetic construct
GGPGHDLLD

SEQ ID NO: 36846 - protein, 9 aa, synthetic construct
GGPGDDYVD

SEQ ID NO: 36847 - protein, 9 aa, synthetic construct
GGPGDDYVT

SEQ ID NO: 36848 - protein, 9 aa, synthetic construct
GGPGDDYYV

SEQ ID NO: 36849 - protein, 9 aa, synthetic construct
GGPGEDIAQ

SEQ ID NO: 36850 - protein, 9 aa, synthetic construct
GGPGEDLFL

SEQ ID NO: 36851 - protein, 9 aa, synthetic construct
GGPGEDLLD

SEQ ID NO: 36852 - protein, 9 aa, synthetic construct
GGPGEDLLG

SEQ ID NO: 36853 - protein, 9 aa, synthetic construct
GGPGEDLLR

SEQ ID NO: 36854 - protein, 9 aa, synthetic construct
GGPGEDQLD

SEQ ID NO: 36855 - protein, 9 aa, synthetic construct
GGPGEDRIR

SEQ ID NO: 36856 - protein, 9 aa, synthetic construct
GGPGEDRIV

SEQ ID NO: 36857 - protein, 9 aa, synthetic construct
GGPGEDRLW

SEQ ID NO: 36858 - protein, 9 aa, synthetic construct
GGPGEDSIL

SEQ ID NO: 36859 - protein, 9 aa, synthetic construct
GGPGEDTIH

SEQ ID NO: 36860 - protein, 9 aa, synthetic construct
GGPGEDTII

SEQ ID NO: 36861 - protein, 9 aa, synthetic construct
GGPGEDTIS

SEQ ID NO: 36862 - protein, 9 aa, synthetic construct
GGPGEDTIT

SEQ ID NO: 36863 - protein, 9 aa, synthetic construct
GGPGEDTLA

SEQ ID NO: 36864 - protein, 9 aa, synthetic construct
GGPGEDTLD

SEQ ID NO: 36865 - protein, 9 aa, synthetic construct
GGPGEDTLI

SEQ ID NO: 36866 - protein, 9 aa, synthetic construct
GGPGEDTVY

SEQ ID NO: 36867 - protein, 9 aa, synthetic construct
GGPGEDVFR

SEQ ID NO: 36868 - protein, 9 aa, synthetic construct
GGPGEDVFV

SEQ ID NO: 36869 - protein, 9 aa, synthetic construct
GGPGEDVLF

SEQ ID NO: 36870 - protein, 9 aa, synthetic construct
GGPGEDVLH

SEQ ID NO: 36871 - protein, 9 aa, synthetic construct
GGPGEDVLI

SEQ ID NO: 36872 - protein, 9 aa, synthetic construct
GGPGEDVLM

SEQ ID NO: 36873 - protein, 9 aa, synthetic construct
GGPGEDVLQ

SEQ ID NO: 36874 - protein, 9 aa, synthetic construct
GGPGEDVLS

SEQ ID NO: 36875 - protein, 9 aa, synthetic construct
GGPGDDYMI

SEQ ID NO: 36876 - protein, 9 aa, synthetic construct
GGPGDDYLY

SEQ ID NO: 36877 - protein, 9 aa, synthetic construct
GGPGDDYLQ

SEQ ID NO: 36878 - protein, 9 aa, synthetic construct
GGPGDDVIG

SEQ ID NO: 36879 - protein, 9 aa, synthetic construct
GGPGDDTMM

SEQ ID NO: 36880 - protein, 9 aa, synthetic construct
GGPGDDTMQ

SEQ ID NO: 36881 - protein, 9 aa, synthetic construct
GGPGDDTMT

SEQ ID NO: 36882 - protein, 9 aa, synthetic construct
GGPGDDTVF

SEQ ID NO: 36883 - protein, 9 aa, synthetic construct
GGPGDDTVY

SEQ ID NO: 36884 - protein, 9 aa, synthetic construct
GGPGDDTYA

SEQ ID NO: 36885 - protein, 9 aa, synthetic construct
GGPGDDTYI

SEQ ID NO: 36886 - protein, 9 aa, synthetic construct
GGPGDDTYM

SEQ ID NO: 36887 - protein, 9 aa, synthetic construct
GGPGDDTYR

SEQ ID NO: 36888 - protein, 9 aa, synthetic construct
GGPGDDTYV

SEQ ID NO: 36889 - protein, 9 aa, synthetic construct
GGPGDDVAF

SEQ ID NO: 36890 - protein, 9 aa, synthetic construct
GGPGDDVFI

SEQ ID NO: 36891 - protein, 9 aa, synthetic construct
GGPGDDVFL

SEQ ID NO: 36892 - protein, 9 aa, synthetic construct
GGPGDDVIN

SEQ ID NO: 36893 - protein, 9 aa, synthetic construct
GGPGDDYLH

SEQ ID NO: 36894 - protein, 9 aa, synthetic construct
GGPGDDVIR

SEQ ID NO: 36895 - protein, 9 aa, synthetic construct
GGPGDDVIY

SEQ ID NO: 36896 - protein, 9 aa, synthetic construct
GGPGDDVLC

SEQ ID NO: 36897 - protein, 9 aa, synthetic construct
GGPGDDVLM

SEQ ID NO: 36898 - protein, 9 aa, synthetic construct
GGPGDDVMD

SEQ ID NO: 36899 - protein, 9 aa, synthetic construct
GGPGDDVMS

SEQ ID NO: 36900 - protein, 9 aa, synthetic construct
GGPGDDVVA

SEQ ID NO: 36901 - protein, 9 aa, synthetic construct
GGPGDDVYH

SEQ ID NO: 36902 - protein, 9 aa, synthetic construct
GGPGDDVYY

SEQ ID NO: 36903 - protein, 9 aa, synthetic construct
GGPGDDWIR

SEQ ID NO: 36904 - protein, 9 aa, synthetic construct
GGPGDDWMR

SEQ ID NO: 36905 - protein, 9 aa, synthetic construct
GGPGDDYID

SEQ ID NO: 36906 - protein, 9 aa, synthetic construct
GGPGDDYLF

SEQ ID NO: 36907 - protein, 9 aa, synthetic construct
GGPGFDDFI

SEQ ID NO: 36908 - protein, 9 aa, synthetic construct
GGPGFDFIL

SEQ ID NO: 36909 - protein, 9 aa, synthetic construct
GGPGFDFLR

SEQ ID NO: 36910 - protein, 9 aa, synthetic construct
GGPGGDVIY

SEQ ID NO: 36911 - protein, 9 aa, synthetic construct
GGPGGDLLY

SEQ ID NO: 36912 - protein, 9 aa, synthetic construct
GGPGGDMLT

SEQ ID NO: 36913 - protein, 9 aa, synthetic construct
GGPGGDRFD

SEQ ID NO: 36914 - protein, 9 aa, synthetic construct
GGPGGDRIV

SEQ ID NO: 36915 - protein, 9 aa, synthetic construct
GGPGGDRLI

SEQ ID NO: 36916 - protein, 9 aa, synthetic construct
GGPGGDSLA

SEQ ID NO: 36917 - protein, 9 aa, synthetic construct
GGPGGDSLT

SEQ ID NO: 36918 - protein, 9 aa, synthetic construct
GGPGGDSLY

SEQ ID NO: 36919 - protein, 9 aa, synthetic construct
GGPGGDTIF

SEQ ID NO: 36920 - protein, 9 aa, synthetic construct
GGPGGDTLD

SEQ ID NO: 36921 - protein, 9 aa, synthetic construct
GGPGGDTLF

SEQ ID NO: 36922 - protein, 9 aa, synthetic construct
GGPGGDTLN

SEQ ID NO: 36923 - protein, 9 aa, synthetic construct
GGPGGDTLS

SEQ ID NO: 36924 - protein, 9 aa, synthetic construct
GGPGGDVLI

SEQ ID NO: 36925 - protein, 9 aa, synthetic construct
GGPGGDLIK

SEQ ID NO: 36926 - protein, 9 aa, synthetic construct
GGPGGDVLR

SEQ ID NO: 36927 - protein, 9 aa, synthetic construct
GGPGGDVLY

SEQ ID NO: 36928 - protein, 9 aa, synthetic construct
GGPGGDWLV

SEQ ID NO: 36929 - protein, 9 aa, synthetic construct
GGPGGDWMH

SEQ ID NO: 36930 - protein, 9 aa, synthetic construct
GGPGGDYLN

SEQ ID NO: 36931 - protein, 9 aa, synthetic construct
GGPGGDYVT

SEQ ID NO: 36932 - protein, 9 aa, synthetic construct
GGPGHDAME

SEQ ID NO: 36933 - protein, 9 aa, synthetic construct
GGPGHDELW

SEQ ID NO: 36934 - protein, 9 aa, synthetic construct
GGPGHDFIN

SEQ ID NO: 36935 - protein, 9 aa, synthetic construct
GGPGHDIIF

SEQ ID NO: 36936 - protein, 9 aa, synthetic construct
GGPGHDILI

SEQ ID NO: 36937 - protein, 9 aa, synthetic construct
GGPGHDILY

SEQ ID NO: 36938 - protein, 9 aa, synthetic construct
GGPGHDLIA

SEQ ID NO: 36939 - protein, 9 aa, synthetic construct
GGPGGDLLW

SEQ ID NO: 36940 - protein, 9 aa, synthetic construct
GGPGGDKID

SEQ ID NO: 36941 - protein, 9 aa, synthetic construct
GGPGFDFLV

SEQ ID NO: 36942 - protein, 9 aa, synthetic construct
GGPGFDTLT

SEQ ID NO: 36943 - protein, 9 aa, synthetic construct
GGPGFDILT

SEQ ID NO: 36944 - protein, 9 aa, synthetic construct
GGPGFDKMI

SEQ ID NO: 36945 - protein, 9 aa, synthetic construct
GGPGFDLAD

SEQ ID NO: 36946 - protein, 9 aa, synthetic construct
GGPGFDLLD

SEQ ID NO: 36947 - protein, 9 aa, synthetic construct
GGPGFDLLI

SEQ ID NO: 36948 - protein, 9 aa, synthetic construct
GGPGFDLLL

SEQ ID NO: 36949 - protein, 9 aa, synthetic construct
GGPGFDNLI

SEQ ID NO: 36950 - protein, 9 aa, synthetic construct
GGPGFDRIF

SEQ ID NO: 36951 - protein, 9 aa, synthetic construct
GGPGFDRLD

SEQ ID NO: 36952 - protein, 9 aa, synthetic construct
GGPGFDRLF

SEQ ID NO: 36953 - protein, 9 aa, synthetic construct
GGPGFDTAA

SEQ ID NO: 36954 - protein, 9 aa, synthetic construct
GGPGFDTLF

SEQ ID NO: 36955 - protein, 9 aa, synthetic construct
GGPGFDTLR

SEQ ID NO: 36956 - protein, 9 aa, synthetic construct
GGPGFDTLV

SEQ ID NO: 36957 - protein, 9 aa, synthetic construct
GGPGGDILF

SEQ ID NO: 36958 - protein, 9 aa, synthetic construct
GGPGFDTLW

SEQ ID NO: 36959 - protein, 9 aa, synthetic construct
GGPGFDTLY

SEQ ID NO: 36960 - protein, 9 aa, synthetic construct
GGPGFDVAK

SEQ ID NO: 36961 - protein, 9 aa, synthetic construct
GGPGFDVIR

SEQ ID NO: 36962 - protein, 9 aa, synthetic construct
GGPGFDVLD

SEQ ID NO: 36963 - protein, 9 aa, synthetic construct
GGPGFDVLK

SEQ ID NO: 36964 - protein, 9 aa, synthetic construct
GGPGFDVVS

SEQ ID NO: 36965 - protein, 9 aa, synthetic construct
GGPGGDAIE

SEQ ID NO: 36966 - protein, 9 aa, synthetic construct
GGPGGDALK

SEQ ID NO: 36967 - protein, 9 aa, synthetic construct
GGPGGDDMR

SEQ ID NO: 36968 - protein, 9 aa, synthetic construct
GGPGGDFLL

SEQ ID NO: 36969 - protein, 9 aa, synthetic construct
GGPGGDHFV

SEQ ID NO: 36970 - protein, 9 aa, synthetic construct
GGPGGDHLN

SEQ ID NO: 36971 - protein, 9 aa, synthetic construct
GGPGNDHLL

SEQ ID NO: 36972 - protein, 9 aa, synthetic construct
GGPGNDHLR

SEQ ID NO: 36973 - protein, 9 aa, synthetic construct
GGPGNDHLW

SEQ ID NO: 36974 - protein, 9 aa, synthetic construct
GGPGQDILG

SEQ ID NO: 36975 - protein, 9 aa, synthetic construct
GGPGRDFLA

SEQ ID NO: 36976 - protein, 9 aa, synthetic construct
GGPGRDFLN

SEQ ID NO: 36977 - protein, 9 aa, synthetic construct
GGPGRDFVR

SEQ ID NO: 36978 - protein, 9 aa, synthetic construct
GGPGRDGMT

SEQ ID NO: 36979 - protein, 9 aa, synthetic construct
GGPGRDHAF

SEQ ID NO: 36980 - protein, 9 aa, synthetic construct
GGPGRDHLK

SEQ ID NO: 36981 - protein, 9 aa, synthetic construct
GGPGRDHLM

SEQ ID NO: 36982 - protein, 9 aa, synthetic construct
GGPGRDHLQ

SEQ ID NO: 36983 - protein, 9 aa, synthetic construct
GGPGRDIAI

SEQ ID NO: 36984 - protein, 9 aa, synthetic construct
GGPGRDIAV

SEQ ID NO: 36985 - protein, 9 aa, synthetic construct
GGPGRDILT

SEQ ID NO: 36986 - protein, 9 aa, synthetic construct
GGPGRDILV

SEQ ID NO: 36987 - protein, 9 aa, synthetic construct
GGPGRDKAW

SEQ ID NO: 36988 - protein, 9 aa, synthetic construct
GGPGRDKLA

SEQ ID NO: 36989 - protein, 9 aa, synthetic construct
GGPGRDKLF

SEQ ID NO: 36990 - protein, 9 aa, synthetic construct
GGPGRDKLS

SEQ ID NO: 36991 - protein, 9 aa, synthetic construct
GGPGRDKLT

SEQ ID NO: 36992 - protein, 9 aa, synthetic construct
GGPGRDKLY

SEQ ID NO: 36993 - protein, 9 aa, synthetic construct
GGPGRDLAH

SEQ ID NO: 36994 - protein, 9 aa, synthetic construct
GGPGRDLIE

SEQ ID NO: 36995 - protein, 9 aa, synthetic construct
GGPGRDLIF

SEQ ID NO: 36996 - protein, 9 aa, synthetic construct
GGPGRDLLA

SEQ ID NO: 36997 - protein, 9 aa, synthetic construct
GGPGRDLLF

SEQ ID NO: 36998 - protein, 9 aa, synthetic construct
GGPGRDLLL

SEQ ID NO: 36999 - protein, 9 aa, synthetic construct
GGPGRDLLR

SEQ ID NO: 37000 - protein, 9 aa, synthetic construct
GGPGRDLLS

SEQ ID NO: 37001 - protein, 9 aa, synthetic construct
GGPGRDLLT

SEQ ID NO: 37002 - protein, 9 aa, synthetic construct
GGPGRDLLY

SEQ ID NO: 37003 - protein, 9 aa, synthetic construct
GGPGRDLMI

SEQ ID NO: 37004 - protein, 9 aa, synthetic construct
GGPGRDFFD

SEQ ID NO: 37005 - protein, 9 aa, synthetic construct
GGPGRDELY

SEQ ID NO: 37006 - protein, 9 aa, synthetic construct
GGPGRDEIQ

SEQ ID NO: 37007 - protein, 9 aa, synthetic construct
GGPGQDTLS

SEQ ID NO: 37008 - protein, 9 aa, synthetic construct
GGPGQDKLW

SEQ ID NO: 37009 - protein, 9 aa, synthetic construct
GGPGQDKVI

SEQ ID NO: 37010 - protein, 9 aa, synthetic construct
GGPGQDLLR

SEQ ID NO: 37011 - protein, 9 aa, synthetic construct
GGPGQDMLN

SEQ ID NO: 37012 - protein, 9 aa, synthetic construct
GGPGQDQII

SEQ ID NO: 37013 - protein, 9 aa, synthetic construct
GGPGQDQLY

SEQ ID NO: 37014 - protein, 9 aa, synthetic construct
GGPGQDQMW

SEQ ID NO: 37015 - protein, 9 aa, synthetic construct
GGPGQDRLE

SEQ ID NO: 37016 - protein, 9 aa, synthetic construct
GGPGQDSLY

SEQ ID NO: 37017 - protein, 9 aa, synthetic construct
GGPGQDTAI

SEQ ID NO: 37018 - protein, 9 aa, synthetic construct
GGPGQDTAL

SEQ ID NO: 37019 - protein, 9 aa, synthetic construct
GGPGQDTFL

SEQ ID NO: 37020 - protein, 9 aa, synthetic construct
GGPGQDTLR

SEQ ID NO: 37021 - protein, 9 aa, synthetic construct
GGPGQDTLW

SEQ ID NO: 37022 - protein, 9 aa, synthetic construct
GGPGRDDLR

SEQ ID NO: 37023 - protein, 9 aa, synthetic construct
GGPGQDTLY

SEQ ID NO: 37024 - protein, 9 aa, synthetic construct
GGPGQDTMF

SEQ ID NO: 37025 - protein, 9 aa, synthetic construct
GGPGQDVFK

SEQ ID NO: 37026 - protein, 9 aa, synthetic construct
GGPGQDVIH

SEQ ID NO: 37027 - protein, 9 aa, synthetic construct
GGPGQDVLY

SEQ ID NO: 37028 - protein, 9 aa, synthetic construct
GGPGQDVYL

SEQ ID NO: 37029 - protein, 9 aa, synthetic construct
GGPGQDWLD

SEQ ID NO: 37030 - protein, 9 aa, synthetic construct
GGPGQDYVN

SEQ ID NO: 37031 - protein, 9 aa, synthetic construct
GGPGRDAFV

SEQ ID NO: 37032 - protein, 9 aa, synthetic construct
GGPGRDALF

SEQ ID NO: 37033 - protein, 9 aa, synthetic construct
GGPGRDALS

SEQ ID NO: 37034 - protein, 9 aa, synthetic construct
GGPGRDALY

SEQ ID NO: 37035 - protein, 9 aa, synthetic construct
GGPGRDDIT

SEQ ID NO: 37036 - protein, 9 aa, synthetic construct
GGPGRDMII

SEQ ID NO: 37037 - protein, 9 aa, synthetic construct
GGPGRDMLV

SEQ ID NO: 37038 - protein, 9 aa, synthetic construct
GGPGRDNIG

SEQ ID NO: 37039 - protein, 9 aa, synthetic construct
GGPGSDFLT

SEQ ID NO: 37040 - protein, 9 aa, synthetic construct
GGPGRDVLT

SEQ ID NO: 37041 - protein, 9 aa, synthetic construct
GGPGRDVLY

SEQ ID NO: 37042 - protein, 9 aa, synthetic construct
GGPGRDVVL

SEQ ID NO: 37043 - protein, 9 aa, synthetic construct
GGPGRDYLD

SEQ ID NO: 37044 - protein, 9 aa, synthetic construct
GGPGRDYLK

SEQ ID NO: 37045 - protein, 9 aa, synthetic construct
GGPGRDYLQ

SEQ ID NO: 37046 - protein, 9 aa, synthetic construct
GGPGRDYLY

SEQ ID NO: 37047 - protein, 9 aa, synthetic construct
GGPGSDAAS

SEQ ID NO: 37048 - protein, 9 aa, synthetic construct
GGPGSDAIA

SEQ ID NO: 37049 - protein, 9 aa, synthetic construct
GGPGSDALW

SEQ ID NO: 37050 - protein, 9 aa, synthetic construct
GGPGSDDIW

SEQ ID NO: 37051 - protein, 9 aa, synthetic construct
GGPGSDELF

SEQ ID NO: 37052 - protein, 9 aa, synthetic construct
GGPGSDFLK

SEQ ID NO: 37053 - protein, 9 aa, synthetic construct
GGPGSDFVF

SEQ ID NO: 37054 - protein, 9 aa, synthetic construct
GGPGRDVLI

SEQ ID NO: 37055 - protein, 9 aa, synthetic construct
GGPGSDHLV

SEQ ID NO: 37056 - protein, 9 aa, synthetic construct
GGPGSDIID

SEQ ID NO: 37057 - protein, 9 aa, synthetic construct
GGPGSDIIT

SEQ ID NO: 37058 - protein, 9 aa, synthetic construct
GGPGSDILI

SEQ ID NO: 37059 - protein, 9 aa, synthetic construct
GGPGSDILL

SEQ ID NO: 37060 - protein, 9 aa, synthetic construct
GGPGSDILS

SEQ ID NO: 37061 - protein, 9 aa, synthetic construct
GGPGSDIYS

SEQ ID NO: 37062 - protein, 9 aa, synthetic construct
GGPGSDLFF

SEQ ID NO: 37063 - protein, 9 aa, synthetic construct
GGPGSDLFV

SEQ ID NO: 37064 - protein, 9 aa, synthetic construct
GGPGSDLIY

SEQ ID NO: 37065 - protein, 9 aa, synthetic construct
GGPGSDLLN

SEQ ID NO: 37066 - protein, 9 aa, synthetic construct
GGPGSDLMF

SEQ ID NO: 37067 - protein, 9 aa, synthetic construct
GGPGSDLYI

SEQ ID NO: 37068 - protein, 9 aa, synthetic construct
GGPGRDVLS

SEQ ID NO: 37069 - protein, 9 aa, synthetic construct
GGPGRDVLH

SEQ ID NO: 37070 - protein, 9 aa, synthetic construct
GGPGRDNIT

SEQ ID NO: 37071 - protein, 9 aa, synthetic construct
GGPGRDTFR

SEQ ID NO: 37072 - protein, 9 aa, synthetic construct
GGPGRDQLF

SEQ ID NO: 37073 - protein, 9 aa, synthetic construct
GGPGRDQLI

SEQ ID NO: 37074 - protein, 9 aa, synthetic construct
GGPGRDQME

SEQ ID NO: 37075 - protein, 9 aa, synthetic construct
GGPGRDQMF

SEQ ID NO: 37076 - protein, 9 aa, synthetic construct
GGPGRDRAQ

SEQ ID NO: 37077 - protein, 9 aa, synthetic construct
GGPGRDRFL

SEQ ID NO: 37078 - protein, 9 aa, synthetic construct
GGPGRDRIY

SEQ ID NO: 37079 - protein, 9 aa, synthetic construct
GGPGRDRLV

SEQ ID NO: 37080 - protein, 9 aa, synthetic construct
GGPGRDRYE

SEQ ID NO: 37081 - protein, 9 aa, synthetic construct
GGPGRDSFV

SEQ ID NO: 37082 - protein, 9 aa, synthetic construct
GGPGRDTAM

SEQ ID NO: 37083 - protein, 9 aa, synthetic construct
GGPGRDTAS

SEQ ID NO: 37084 - protein, 9 aa, synthetic construct
GGPGRDTAV

SEQ ID NO: 37085 - protein, 9 aa, synthetic construct
GGPGRDTID

SEQ ID NO: 37086 - protein, 9 aa, synthetic construct
GGPGRDVLD

SEQ ID NO: 37087 - protein, 9 aa, synthetic construct
GGPGRDTIY

SEQ ID NO: 37088 - protein, 9 aa, synthetic construct
GGPGRDTLN

SEQ ID NO: 37089 - protein, 9 aa, synthetic construct
GGPGRDTLS

SEQ ID NO: 37090 - protein, 9 aa, synthetic construct
GGPGRDTLT

SEQ ID NO: 37091 - protein, 9 aa, synthetic construct
GGPGRDTLV

SEQ ID NO: 37092 - protein, 9 aa, synthetic construct
GGPGRDTLY

SEQ ID NO: 37093 - protein, 9 aa, synthetic construct
GGPGRDTMF

SEQ ID NO: 37094 - protein, 9 aa, synthetic construct
GGPGRDTMS

SEQ ID NO: 37095 - protein, 9 aa, synthetic construct
GGPGRDTMT

SEQ ID NO: 37096 - protein, 9 aa, synthetic construct
GGPGRDTVS

SEQ ID NO: 37097 - protein, 9 aa, synthetic construct
GGPGRDVFI

SEQ ID NO: 37098 - protein, 9 aa, synthetic construct
GGPGRDVIE

SEQ ID NO: 37099 - protein, 9 aa, synthetic construct
GGPGRDVIR

SEQ ID NO: 37100 - protein, 9 aa, synthetic construct
GGPGQDKLR

SEQ ID NO: 37101 - protein, 9 aa, synthetic construct
GGPGQDHLF

SEQ ID NO: 37102 - protein, 9 aa, synthetic construct
GGPGNDIFV

SEQ ID NO: 37103 - protein, 9 aa, synthetic construct
GGPGQDFVR

SEQ ID NO: 37104 - protein, 9 aa, synthetic construct
GGPGNDNLF

SEQ ID NO: 37105 - protein, 9 aa, synthetic construct
GGPGNDNLG

SEQ ID NO: 37106 - protein, 9 aa, synthetic construct
GGPGNDNLV

SEQ ID NO: 37107 - protein, 9 aa, synthetic construct
GGPGNDNMD

SEQ ID NO: 37108 - protein, 9 aa, synthetic construct
GGPGNDQIQ

SEQ ID NO: 37109 - protein, 9 aa, synthetic construct
GGPGNDQLY

SEQ ID NO: 37110 - protein, 9 aa, synthetic construct
GGPGNDQMF

SEQ ID NO: 37111 - protein, 9 aa, synthetic construct
GGPGNDQVV

SEQ ID NO: 37112 - protein, 9 aa, synthetic construct
GGPGNDRIE

SEQ ID NO: 37113 - protein, 9 aa, synthetic construct
GGPGNDRIV

SEQ ID NO: 37114 - protein, 9 aa, synthetic construct
GGPGNDRLA

SEQ ID NO: 37115 - protein, 9 aa, synthetic construct
GGPGNDRLR

SEQ ID NO: 37116 - protein, 9 aa, synthetic construct
GGPGNDRLV

SEQ ID NO: 37117 - protein, 9 aa, synthetic construct
GGPGNDRMA

SEQ ID NO: 37118 - protein, 9 aa, synthetic construct
GGPGNDRMD

SEQ ID NO: 37119 - protein, 9 aa, synthetic construct
GGPGNDRME

SEQ ID NO: 37120 - protein, 9 aa, synthetic construct
GGPGNDRMH

SEQ ID NO: 37121 - protein, 9 aa, synthetic construct
GGPGNDRMM

SEQ ID NO: 37122 - protein, 9 aa, synthetic construct
GGPGNDRMR

SEQ ID NO: 37123 - protein, 9 aa, synthetic construct
GGPGNDRVN

SEQ ID NO: 37124 - protein, 9 aa, synthetic construct
GGPGNDRYR

SEQ ID NO: 37125 - protein, 9 aa, synthetic construct
GGPGNDSFS

SEQ ID NO: 37126 - protein, 9 aa, synthetic construct
GGPGNDSIA

SEQ ID NO: 37127 - protein, 9 aa, synthetic construct
GGPGNDSID

SEQ ID NO: 37128 - protein, 9 aa, synthetic construct
GGPGNDSIL

SEQ ID NO: 37129 - protein, 9 aa, synthetic construct
GGPGNDSIW

SEQ ID NO: 37130 - protein, 9 aa, synthetic construct
GGPGNDSIY

SEQ ID NO: 37131 - protein, 9 aa, synthetic construct
GGPGNDSLA

SEQ ID NO: 37132 - protein, 9 aa, synthetic construct
GGPGNDSLM

SEQ ID NO: 37133 - protein, 9 aa, synthetic construct
GGPGNDNLD

SEQ ID NO: 37134 - protein, 9 aa, synthetic construct
GGPGNDNLA

SEQ ID NO: 37135 - protein, 9 aa, synthetic construct
GGPGNDNIL

SEQ ID NO: 37136 - protein, 9 aa, synthetic construct
GGPGNDLIL

SEQ ID NO: 37137 - protein, 9 aa, synthetic construct
GGPGNDIID

SEQ ID NO: 37138 - protein, 9 aa, synthetic construct
GGPGNDIIS

SEQ ID NO: 37139 - protein, 9 aa, synthetic construct
GGPGNDILF

SEQ ID NO: 37140 - protein, 9 aa, synthetic construct
GGPGNDILK

SEQ ID NO: 37141 - protein, 9 aa, synthetic construct
GGPGNDIMD

SEQ ID NO: 37142 - protein, 9 aa, synthetic construct
GGPGNDIVF

SEQ ID NO: 37143 - protein, 9 aa, synthetic construct
GGPGNDIYL

SEQ ID NO: 37144 - protein, 9 aa, synthetic construct
GGPGNDKIE

SEQ ID NO: 37145 - protein, 9 aa, synthetic construct
GGPGNDKIW

SEQ ID NO: 37146 - protein, 9 aa, synthetic construct
GGPGNDKLL

SEQ ID NO: 37147 - protein, 9 aa, synthetic construct
GGPGNDKLS

SEQ ID NO: 37148 - protein, 9 aa, synthetic construct
GGPGNDLFA

SEQ ID NO: 37149 - protein, 9 aa, synthetic construct
GGPGNDLIA

SEQ ID NO: 37150 - protein, 9 aa, synthetic construct
GGPGNDLLA

SEQ ID NO: 37151 - protein, 9 aa, synthetic construct
GGPGNDNID

SEQ ID NO: 37152 - protein, 9 aa, synthetic construct
GGPGNDLLF

SEQ ID NO: 37153 - protein, 9 aa, synthetic construct
GGPGNDLLG

SEQ ID NO: 37154 - protein, 9 aa, synthetic construct
GGPGNDLLL

SEQ ID NO: 37155 - protein, 9 aa, synthetic construct
GGPGNDLLN

SEQ ID NO: 37156 - protein, 9 aa, synthetic construct
GGPGNDLLY

SEQ ID NO: 37157 - protein, 9 aa, synthetic construct
GGPGNDLME

SEQ ID NO: 37158 - protein, 9 aa, synthetic construct
GGPGNDLMS

SEQ ID NO: 37159 - protein, 9 aa, synthetic construct
GGPGNDLVI

SEQ ID NO: 37160 - protein, 9 aa, synthetic construct
GGPGNDLYW

SEQ ID NO: 37161 - protein, 9 aa, synthetic construct
GGPGNDMID

SEQ ID NO: 37162 - protein, 9 aa, synthetic construct
GGPGNDMIH

SEQ ID NO: 37163 - protein, 9 aa, synthetic construct
GGPGNDMIV

SEQ ID NO: 37164 - protein, 9 aa, synthetic construct
GGPGNDMLS

SEQ ID NO: 37165 - protein, 9 aa, synthetic construct
GGPGNDSLQ

SEQ ID NO: 37166 - protein, 9 aa, synthetic construct
GGPGNDSMK

SEQ ID NO: 37167 - protein, 9 aa, synthetic construct
GGPGNDTAE

SEQ ID NO: 37168 - protein, 9 aa, synthetic construct
GGPGPDLFY

SEQ ID NO: 37169 - protein, 9 aa, synthetic construct
GGPGNDWLR

SEQ ID NO: 37170 - protein, 9 aa, synthetic construct
GGPGNDYIS

SEQ ID NO: 37171 - protein, 9 aa, synthetic construct
GGPGNDYLH

SEQ ID NO: 37172 - protein, 9 aa, synthetic construct
GGPGNDYLK

SEQ ID NO: 37173 - protein, 9 aa, synthetic construct
GGPGNDYLS

SEQ ID NO: 37174 - protein, 9 aa, synthetic construct
GGPGNDYLV

SEQ ID NO: 37175 - protein, 9 aa, synthetic construct
GGPGNDYMR

SEQ ID NO: 37176 - protein, 9 aa, synthetic construct
GGPGNDYVY

SEQ ID NO: 37177 - protein, 9 aa, synthetic construct
GGPGPDALD

SEQ ID NO: 37178 - protein, 9 aa, synthetic construct
GGPGPDALS

SEQ ID NO: 37179 - protein, 9 aa, synthetic construct
GGPGPDFLF

SEQ ID NO: 37180 - protein, 9 aa, synthetic construct
GGPGPDHLI

SEQ ID NO: 37181 - protein, 9 aa, synthetic construct
GGPGPDKMF

SEQ ID NO: 37182 - protein, 9 aa, synthetic construct
GGPGPDLLF

SEQ ID NO: 37183 - protein, 9 aa, synthetic construct
GGPGNDWLH

SEQ ID NO: 37184 - protein, 9 aa, synthetic construct
GGPGPDLLR

SEQ ID NO: 37185 - protein, 9 aa, synthetic construct
GGPGPDLLY

SEQ ID NO: 37186 - protein, 9 aa, synthetic construct
GGPGPDQLR

SEQ ID NO: 37187 - protein, 9 aa, synthetic construct
GGPGPDRLR

SEQ ID NO: 37188 - protein, 9 aa, synthetic construct
GGPGPDTFV

SEQ ID NO: 37189 - protein, 9 aa, synthetic construct
GGPGPDTLR

SEQ ID NO: 37190 - protein, 9 aa, synthetic construct
GGPGPDTLY

SEQ ID NO: 37191 - protein, 9 aa, synthetic construct
GGPGPDVIF

SEQ ID NO: 37192 - protein, 9 aa, synthetic construct
GGPGPDVLI

SEQ ID NO: 37193 - protein, 9 aa, synthetic construct
GGPGPDVLN

SEQ ID NO: 37194 - protein, 9 aa, synthetic construct
GGPGPDXLF

SEQ ID NO: 37195 - protein, 9 aa, synthetic construct
GGPGQDEIT

SEQ ID NO: 37196 - protein, 9 aa, synthetic construct
GGPGQDFLD

SEQ ID NO: 37197 - protein, 9 aa, synthetic construct
GGPGNDWLQ

SEQ ID NO: 37198 - protein, 9 aa, synthetic construct
GGPGNDWLF

SEQ ID NO: 37199 - protein, 9 aa, synthetic construct
GGPGNDTAL

SEQ ID NO: 37200 - protein, 9 aa, synthetic construct
GGPGNDTVS

SEQ ID NO: 37201 - protein, 9 aa, synthetic construct
GGPGNDTFV

SEQ ID NO: 37202 - protein, 9 aa, synthetic construct
GGPGNDTIA

SEQ ID NO: 37203 - protein, 9 aa, synthetic construct
GGPGNDTIG

SEQ ID NO: 37204 - protein, 9 aa, synthetic construct
GGPGNDTIM

SEQ ID NO: 37205 - protein, 9 aa, synthetic construct
GGPGNDTIQ

SEQ ID NO: 37206 - protein, 9 aa, synthetic construct
GGPGNDTLM

SEQ ID NO: 37207 - protein, 9 aa, synthetic construct
GGPGNDTLW

SEQ ID NO: 37208 - protein, 9 aa, synthetic construct
GGPGNDTMD

SEQ ID NO: 37209 - protein, 9 aa, synthetic construct
GGPGNDTMH

SEQ ID NO: 37210 - protein, 9 aa, synthetic construct
GGPGNDTMI

SEQ ID NO: 37211 - protein, 9 aa, synthetic construct
GGPGNDTML

SEQ ID NO: 37212 - protein, 9 aa, synthetic construct
GGPGNDTMM

SEQ ID NO: 37213 - protein, 9 aa, synthetic construct
GGPGNDTMT

SEQ ID NO: 37214 - protein, 9 aa, synthetic construct
GGPGNDTVV

SEQ ID NO: 37215 - protein, 9 aa, synthetic construct
GGPGNDVYV

SEQ ID NO: 37216 - protein, 9 aa, synthetic construct
GGPGNDTYY

SEQ ID NO: 37217 - protein, 9 aa, synthetic construct
GGPGNDVII

SEQ ID NO: 37218 - protein, 9 aa, synthetic construct
GGPGNDVIN

SEQ ID NO: 37219 - protein, 9 aa, synthetic construct
GGPGNDVIR

SEQ ID NO: 37220 - protein, 9 aa, synthetic construct
GGPGNDVLS

SEQ ID NO: 37221 - protein, 9 aa, synthetic construct
GGPGNDVMI

SEQ ID NO: 37222 - protein, 9 aa, synthetic construct
GGPGNDVML

SEQ ID NO: 37223 - protein, 9 aa, synthetic construct
GGPGNDVMS

SEQ ID NO: 37224 - protein, 9 aa, synthetic construct
GGPGNDVVA

SEQ ID NO: 37225 - protein, 9 aa, synthetic construct
GGPGNDVVE

SEQ ID NO: 37226 - protein, 9 aa, synthetic construct
GGPGNDVVQ

SEQ ID NO: 37227 - protein, 9 aa, synthetic construct
GGPGNDVYR

SEQ ID NO: 37228 - protein, 9 aa, synthetic construct
GGPGNDVYT

SEQ ID NO: 37229 - protein, 9 aa, synthetic construct
GGQGHDVLT

SEQ ID NO: 37230 - protein, 9 aa, synthetic construct
GGQGIDAIR

SEQ ID NO: 37231 - protein, 9 aa, synthetic construct
GGRGMDTLQ

SEQ ID NO: 37232 - protein, 9 aa, synthetic construct
GGRGDDLII

SEQ ID NO: 37233 - protein, 9 aa, synthetic construct
GGRGDDFVE

SEQ ID NO: 37234 - protein, 9 aa, synthetic construct
GGRGDDFVN

SEQ ID NO: 37235 - protein, 9 aa, synthetic construct
GGRGDDFVS

SEQ ID NO: 37236 - protein, 9 aa, synthetic construct
GGRGDDFYI

SEQ ID NO: 37237 - protein, 9 aa, synthetic construct
GGRGDDGIS

SEQ ID NO: 37238 - protein, 9 aa, synthetic construct
GGRGDDGLD

SEQ ID NO: 37239 - protein, 9 aa, synthetic construct
GGRGDDGYI

SEQ ID NO: 37240 - protein, 9 aa, synthetic construct
GGRGDDGYL

SEQ ID NO: 37241 - protein, 9 aa, synthetic construct
GGRGDDHLN

SEQ ID NO: 37242 - protein, 9 aa, synthetic construct
GGRGDDHLS

SEQ ID NO: 37243 - protein, 9 aa, synthetic construct
GGRGDDHVE

SEQ ID NO: 37244 - protein, 9 aa, synthetic construct
GGRGDDHVL

SEQ ID NO: 37245 - protein, 9 aa, synthetic construct
GGRGDDIAH

SEQ ID NO: 37246 - protein, 9 aa, synthetic construct
GGRGDDIAY

SEQ ID NO: 37247 - protein, 9 aa, synthetic construct
GGRGDDIFY

SEQ ID NO: 37248 - protein, 9 aa, synthetic construct
GGRGDDIID

SEQ ID NO: 37249 - protein, 9 aa, synthetic construct
GGRGDDIIR

SEQ ID NO: 37250 - protein, 9 aa, synthetic construct
GGRGDDIIS

SEQ ID NO: 37251 - protein, 9 aa, synthetic construct
GGRGDDIIY

SEQ ID NO: 37252 - protein, 9 aa, synthetic construct
GGRGDDILQ

SEQ ID NO: 37253 - protein, 9 aa, synthetic construct
GGRGDDIMT

SEQ ID NO: 37254 - protein, 9 aa, synthetic construct
GGRGDDIVW

SEQ ID NO: 37255 - protein, 9 aa, synthetic construct
GGRGDDIYR

SEQ ID NO: 37256 - protein, 9 aa, synthetic construct
GGRGDDKIE

SEQ ID NO: 37257 - protein, 9 aa, synthetic construct
GGRGDDKIS

SEQ ID NO: 37258 - protein, 9 aa, synthetic construct
GGRGDDKLD

SEQ ID NO: 37259 - protein, 9 aa, synthetic construct
GGRGDDKLY

SEQ ID NO: 37260 - protein, 9 aa, synthetic construct
GGRGDDLAG

SEQ ID NO: 37261 - protein, 9 aa, synthetic construct
GGRGDDLFL

SEQ ID NO: 37262 - protein, 9 aa, synthetic construct
GGRGDDFMK

SEQ ID NO: 37263 - protein, 9 aa, synthetic construct
GGRGDDFMF

SEQ ID NO: 37264 - protein, 9 aa, synthetic construct
GGRGDDFLY

SEQ ID NO: 37265 - protein, 9 aa, synthetic construct
GGRGDDELR

SEQ ID NO: 37266 - protein, 9 aa, synthetic construct
GGRGDDDLF

SEQ ID NO: 37267 - protein, 9 aa, synthetic construct
GGRGDDDLI

SEQ ID NO: 37268 - protein, 9 aa, synthetic construct
GGRGDDDLK

SEQ ID NO: 37269 - protein, 9 aa, synthetic construct
GGRGDDDLN

SEQ ID NO: 37270 - protein, 9 aa, synthetic construct
GGRGDDDLY

SEQ ID NO: 37271 - protein, 9 aa, synthetic construct
GGRGDDEIA

SEQ ID NO: 37272 - protein, 9 aa, synthetic construct
GGRGDDEIL

SEQ ID NO: 37273 - protein, 9 aa, synthetic construct
GGRGDDEIN

SEQ ID NO: 37274 - protein, 9 aa, synthetic construct
GGRGDDEIR

SEQ ID NO: 37275 - protein, 9 aa, synthetic construct
GGRGDDEIS

SEQ ID NO: 37276 - protein, 9 aa, synthetic construct
GGRGDDEIW

SEQ ID NO: 37277 - protein, 9 aa, synthetic construct
GGRGDDELF

SEQ ID NO: 37278 - protein, 9 aa, synthetic construct
GGRGDDELK

SEQ ID NO: 37279 - protein, 9 aa, synthetic construct
GGRGDDELT

SEQ ID NO: 37280 - protein, 9 aa, synthetic construct
GGRGDDFLS

SEQ ID NO: 37281 - protein, 9 aa, synthetic construct
GGRGDDELW

SEQ ID NO: 37282 - protein, 9 aa, synthetic construct
GGRGDDEMH

SEQ ID NO: 37283 - protein, 9 aa, synthetic construct
GGRGDDEMS

SEQ ID NO: 37284 - protein, 9 aa, synthetic construct
GGRGDDEVA

SEQ ID NO: 37285 - protein, 9 aa, synthetic construct
GGRGDDEVY

SEQ ID NO: 37286 - protein, 9 aa, synthetic construct
GGRGDDFIE

SEQ ID NO: 37287 - protein, 9 aa, synthetic construct
GGRGDDFIH

SEQ ID NO: 37288 - protein, 9 aa, synthetic construct
GGRGDDFIR

SEQ ID NO: 37289 - protein, 9 aa, synthetic construct
GGRGDDFIT

SEQ ID NO: 37290 - protein, 9 aa, synthetic construct
GGRGDDFLG

SEQ ID NO: 37291 - protein, 9 aa, synthetic construct
GGRGDDFLI

SEQ ID NO: 37292 - protein, 9 aa, synthetic construct
GGRGDDFLL

SEQ ID NO: 37293 - protein, 9 aa, synthetic construct
GGRGDDFLR

SEQ ID NO: 37294 - protein, 9 aa, synthetic construct
GGRGDDLID

SEQ ID NO: 37295 - protein, 9 aa, synthetic construct
GGRGDDLIT

SEQ ID NO: 37296 - protein, 9 aa, synthetic construct
GGRGDDSVF

SEQ ID NO: 37297 - protein, 9 aa, synthetic construct
GGRGDDLIY

SEQ ID NO: 37298 - protein, 9 aa, synthetic construct
GGRGDDQMD

SEQ ID NO: 37299 - protein, 9 aa, synthetic construct
GGRGDDQMF

SEQ ID NO: 37300 - protein, 9 aa, synthetic construct
GGRGDDQYV

SEQ ID NO: 37301 - protein, 9 aa, synthetic construct
GGRGDDRAE

SEQ ID NO: 37302 - protein, 9 aa, synthetic construct
GGRGDDRAY

SEQ ID NO: 37303 - protein, 9 aa, synthetic construct
GGRGDDRFS

SEQ ID NO: 37304 - protein, 9 aa, synthetic construct
GGRGDDRIA

SEQ ID NO: 37305 - protein, 9 aa, synthetic construct
GGRGDDRID

SEQ ID NO: 37306 - protein, 9 aa, synthetic construct
GGRGDDRIG

SEQ ID NO: 37307 - protein, 9 aa, synthetic construct
GGRGDDRIH

SEQ ID NO: 37308 - protein, 9 aa, synthetic construct
GGRGDDRIL

SEQ ID NO: 37309 - protein, 9 aa, synthetic construct
GGRGDDRIN

SEQ ID NO: 37310 - protein, 9 aa, synthetic construct
GGRGDDRIT

SEQ ID NO: 37311 - protein, 9 aa, synthetic construct
GGRGDDRIW

SEQ ID NO: 37312 - protein, 9 aa, synthetic construct
GGRGDDRLH

SEQ ID NO: 37313 - protein, 9 aa, synthetic construct
GGRGDDRLM

SEQ ID NO: 37314 - protein, 9 aa, synthetic construct
GGRGDDRMA

SEQ ID NO: 37315 - protein, 9 aa, synthetic construct
GGRGDDRMD

SEQ ID NO: 37316 - protein, 9 aa, synthetic construct
GGRGDDRMR

SEQ ID NO: 37317 - protein, 9 aa, synthetic construct
GGRGDDRVE

SEQ ID NO: 37318 - protein, 9 aa, synthetic construct
GGRGDDRVF

SEQ ID NO: 37319 - protein, 9 aa, synthetic construct
GGRGDDRVH

SEQ ID NO: 37320 - protein, 9 aa, synthetic construct
GGRGDDRVL

SEQ ID NO: 37321 - protein, 9 aa, synthetic construct
GGRGDDSFI

SEQ ID NO: 37322 - protein, 9 aa, synthetic construct
GGRGDDSIN

SEQ ID NO: 37323 - protein, 9 aa, synthetic construct
GGRGDDSIW

SEQ ID NO: 37324 - protein, 9 aa, synthetic construct
GGRGDDSLG

SEQ ID NO: 37325 - protein, 9 aa, synthetic construct
GGRGDDSLH

SEQ ID NO: 37326 - protein, 9 aa, synthetic construct
GGRGDDSMS

SEQ ID NO: 37327 - protein, 9 aa, synthetic construct
GGRGDDQIN

SEQ ID NO: 37328 - protein, 9 aa, synthetic construct
GGRGDDQFD

SEQ ID NO: 37329 - protein, 9 aa, synthetic construct
GGRGDDNLY

SEQ ID NO: 37330 - protein, 9 aa, synthetic construct
GGRGDDMIA

SEQ ID NO: 37331 - protein, 9 aa, synthetic construct
GGRGDDLLF

SEQ ID NO: 37332 - protein, 9 aa, synthetic construct
GGRGDDLLG

SEQ ID NO: 37333 - protein, 9 aa, synthetic construct
GGRGDDLLM

SEQ ID NO: 37334 - protein, 9 aa, synthetic construct
GGRGDDLMA

SEQ ID NO: 37335 - protein, 9 aa, synthetic construct
GGRGDDLMF

SEQ ID NO: 37336 - protein, 9 aa, synthetic construct
GGRGDDLMG

SEQ ID NO: 37337 - protein, 9 aa, synthetic construct
GGRGDDLMR

SEQ ID NO: 37338 - protein, 9 aa, synthetic construct
GGRGDDLVA

SEQ ID NO: 37339 - protein, 9 aa, synthetic construct
GGRGDDLVD

SEQ ID NO: 37340 - protein, 9 aa, synthetic construct
GGRGDDLVE

SEQ ID NO: 37341 - protein, 9 aa, synthetic construct
GGRGDDLVV

SEQ ID NO: 37342 - protein, 9 aa, synthetic construct
GGRGDDLYH

SEQ ID NO: 37343 - protein, 9 aa, synthetic construct
GGRGDDLYI

SEQ ID NO: 37344 - protein, 9 aa, synthetic construct
GGRGDDMIR

SEQ ID NO: 37345 - protein, 9 aa, synthetic construct
GGRGDDNLT

SEQ ID NO: 37346 - protein, 9 aa, synthetic construct
GGRGDDMIS

SEQ ID NO: 37347 - protein, 9 aa, synthetic construct
GGRGDDMLA

SEQ ID NO: 37348 - protein, 9 aa, synthetic construct
GGRGDDMLF

SEQ ID NO: 37349 - protein, 9 aa, synthetic construct
GGRGDDMLK

SEQ ID NO: 37350 - protein, 9 aa, synthetic construct
GGRGDDMLL

SEQ ID NO: 37351 - protein, 9 aa, synthetic construct
GGRGDDMLN

SEQ ID NO: 37352 - protein, 9 aa, synthetic construct
GGRGDDMLS

SEQ ID NO: 37353 - protein, 9 aa, synthetic construct
GGRGDDNIE

SEQ ID NO: 37354 - protein, 9 aa, synthetic construct
GGRGDDNIG

SEQ ID NO: 37355 - protein, 9 aa, synthetic construct
GGRGDDNIN

SEQ ID NO: 37356 - protein, 9 aa, synthetic construct
GGRGDDNIY

SEQ ID NO: 37357 - protein, 9 aa, synthetic construct
GGRGDDNLG

SEQ ID NO: 37358 - protein, 9 aa, synthetic construct
GGRGDDNLS

SEQ ID NO: 37359 - protein, 9 aa, synthetic construct
GGRGDDDII

SEQ ID NO: 37360 - protein, 9 aa, synthetic construct
GGRGDDDIE

SEQ ID NO: 37361 - protein, 9 aa, synthetic construct
GGRGDDAYL

SEQ ID NO: 37362 - protein, 9 aa, synthetic construct
GGRGDDAVQ

SEQ ID NO: 37363 - protein, 9 aa, synthetic construct
GGRGADKLG

SEQ ID NO: 37364 - protein, 9 aa, synthetic construct
GGRGADKLS

SEQ ID NO: 37365 - protein, 9 aa, synthetic construct
GGRGADKLY

SEQ ID NO: 37366 - protein, 9 aa, synthetic construct
GGRGADLFF

SEQ ID NO: 37367 - protein, 9 aa, synthetic construct
GGRGADLLE

SEQ ID NO: 37368 - protein, 9 aa, synthetic construct
GGRGADLLG

SEQ ID NO: 37369 - protein, 9 aa, synthetic construct
GGRGADLLL

SEQ ID NO: 37370 - protein, 9 aa, synthetic construct
GGRGADLMI

SEQ ID NO: 37371 - protein, 9 aa, synthetic construct
GGRGADLMQ

SEQ ID NO: 37372 - protein, 9 aa, synthetic construct
GGRGADLMV

SEQ ID NO: 37373 - protein, 9 aa, synthetic construct
GGRGADLVA

SEQ ID NO: 37374 - protein, 9 aa, synthetic construct
GGRGADLVE

SEQ ID NO: 37375 - protein, 9 aa, synthetic construct
GGRGADMLE

SEQ ID NO: 37376 - protein, 9 aa, synthetic construct
GGRGADMLM

SEQ ID NO: 37377 - protein, 9 aa, synthetic construct
GGRGADNLT

SEQ ID NO: 37378 - protein, 9 aa, synthetic construct
GGRGADQIF

SEQ ID NO: 37379 - protein, 9 aa, synthetic construct
GGRGADQIR

SEQ ID NO: 37380 - protein, 9 aa, synthetic construct
GGRGADQIV

SEQ ID NO: 37381 - protein, 9 aa, synthetic construct
GGRGADQLD

SEQ ID NO: 37382 - protein, 9 aa, synthetic construct
GGRGADQLF

SEQ ID NO: 37383 - protein, 9 aa, synthetic construct
GGRGADQLS

SEQ ID NO: 37384 - protein, 9 aa, synthetic construct
GGRGADQLV

SEQ ID NO: 37385 - protein, 9 aa, synthetic construct
GGRGADQMK

SEQ ID NO: 37386 - protein, 9 aa, synthetic construct
GGRGADRFD

SEQ ID NO: 37387 - protein, 9 aa, synthetic construct
GGRGADRFF

SEQ ID NO: 37388 - protein, 9 aa, synthetic construct
GGRGADRFN

SEQ ID NO: 37389 - protein, 9 aa, synthetic construct
GGRGADRIF

SEQ ID NO: 37390 - protein, 9 aa, synthetic construct
GGRGADRII

SEQ ID NO: 37391 - protein, 9 aa, synthetic construct
GGRGADRIR

SEQ ID NO: 37392 - protein, 9 aa, synthetic construct
GGRGADKIY

SEQ ID NO: 37393 - protein, 9 aa, synthetic construct
GGRGADKIK

SEQ ID NO: 37394 - protein, 9 aa, synthetic construct
GGRGADIYF

SEQ ID NO: 37395 - protein, 9 aa, synthetic construct
GGRGADEFH

SEQ ID NO: 37396 - protein, 9 aa, synthetic construct
GGRGADAFI

SEQ ID NO: 37397 - protein, 9 aa, synthetic construct
GGRGADAIS

SEQ ID NO: 37398 - protein, 9 aa, synthetic construct
GGRGADALD

SEQ ID NO: 37399 - protein, 9 aa, synthetic construct
GGRGADALY

SEQ ID NO: 37400 - protein, 9 aa, synthetic construct
GGRGADAVQ

SEQ ID NO: 37401 - protein, 9 aa, synthetic construct
GGRGADAVS

SEQ ID NO: 37402 - protein, 9 aa, synthetic construct
GGRGADDIS

SEQ ID NO: 37403 - protein, 9 aa, synthetic construct
GGRGADDLA

SEQ ID NO: 37404 - protein, 9 aa, synthetic construct
GGRGADDLD

SEQ ID NO: 37405 - protein, 9 aa, synthetic construct
GGRGADDLF

SEQ ID NO: 37406 - protein, 9 aa, synthetic construct
GGRGADDLH

SEQ ID NO: 37407 - protein, 9 aa, synthetic construct
GGRGADDLL

SEQ ID NO: 37408 - protein, 9 aa, synthetic construct
GGRGADDMA

SEQ ID NO: 37409 - protein, 9 aa, synthetic construct
GGRGADEIH

SEQ ID NO: 37410 - protein, 9 aa, synthetic construct
GGRGADIYE

SEQ ID NO: 37411 - protein, 9 aa, synthetic construct
GGRGADEIQ

SEQ ID NO: 37412 - protein, 9 aa, synthetic construct
GGRGADELS

SEQ ID NO: 37413 - protein, 9 aa, synthetic construct
GGRGADELV

SEQ ID NO: 37414 - protein, 9 aa, synthetic construct
GGRGADFLQ

SEQ ID NO: 37415 - protein, 9 aa, synthetic construct
GGRGADFLY

SEQ ID NO: 37416 - protein, 9 aa, synthetic construct
GGRGADHLA

SEQ ID NO: 37417 - protein, 9 aa, synthetic construct
GGRGADHLI

SEQ ID NO: 37418 - protein, 9 aa, synthetic construct
GGRGADIAR

SEQ ID NO: 37419 - protein, 9 aa, synthetic construct
GGRGADIAV

SEQ ID NO: 37420 - protein, 9 aa, synthetic construct
GGRGADILE

SEQ ID NO: 37421 - protein, 9 aa, synthetic construct
GGRGADILH

SEQ ID NO: 37422 - protein, 9 aa, synthetic construct
GGRGADILM

SEQ ID NO: 37423 - protein, 9 aa, synthetic construct
GGRGADILY

SEQ ID NO: 37424 - protein, 9 aa, synthetic construct
GGRGADRLQ

SEQ ID NO: 37425 - protein, 9 aa, synthetic construct
GGRGADRML

SEQ ID NO: 37426 - protein, 9 aa, synthetic construct
GGRGADRMV

SEQ ID NO: 37427 - protein, 9 aa, synthetic construct
GGRGADYLH

SEQ ID NO: 37428 - protein, 9 aa, synthetic construct
GGRGADVLF

SEQ ID NO: 37429 - protein, 9 aa, synthetic construct
GGRGADVLI

SEQ ID NO: 37430 - protein, 9 aa, synthetic construct
GGRGADVME

SEQ ID NO: 37431 - protein, 9 aa, synthetic construct
GGRGADVMS

SEQ ID NO: 37432 - protein, 9 aa, synthetic construct
GGRGADVMV

SEQ ID NO: 37433 - protein, 9 aa, synthetic construct
GGRGADVVD

SEQ ID NO: 37434 - protein, 9 aa, synthetic construct
GGRGADVVF

SEQ ID NO: 37435 - protein, 9 aa, synthetic construct
GGRGADVVL

SEQ ID NO: 37436 - protein, 9 aa, synthetic construct
GGRGADVVN

SEQ ID NO: 37437 - protein, 9 aa, synthetic construct
GGRGADWIL

SEQ ID NO: 37438 - protein, 9 aa, synthetic construct
GGRGADWLE

SEQ ID NO: 37439 - protein, 9 aa, synthetic construct
GGRGADYFV

SEQ ID NO: 37440 - protein, 9 aa, synthetic construct
GGRGADYLD

SEQ ID NO: 37441 - protein, 9 aa, synthetic construct
GGRGADYLI

SEQ ID NO: 37442 - protein, 9 aa, synthetic construct
GGRGADVIN

SEQ ID NO: 37443 - protein, 9 aa, synthetic construct
GGRGADYME

SEQ ID NO: 37444 - protein, 9 aa, synthetic construct
GGRGCDDIS

SEQ ID NO: 37445 - protein, 9 aa, synthetic construct
GGRGCDSIS

SEQ ID NO: 37446 - protein, 9 aa, synthetic construct
GGRGDDAIE

SEQ ID NO: 37447 - protein, 9 aa, synthetic construct
GGRGDDAIQ

SEQ ID NO: 37448 - protein, 9 aa, synthetic construct
GGRGDDAIV

SEQ ID NO: 37449 - protein, 9 aa, synthetic construct
GGRGDDALD

SEQ ID NO: 37450 - protein, 9 aa, synthetic construct
GGRGDDALF

SEQ ID NO: 37451 - protein, 9 aa, synthetic construct
GGRGDDALK

SEQ ID NO: 37452 - protein, 9 aa, synthetic construct
GGRGDDALR

SEQ ID NO: 37453 - protein, 9 aa, synthetic construct
GGRGDDALT

SEQ ID NO: 37454 - protein, 9 aa, synthetic construct
GGRGDDAMT

SEQ ID NO: 37455 - protein, 9 aa, synthetic construct
GGRGDDAVL

SEQ ID NO: 37456 - protein, 9 aa, synthetic construct
GGRGADVIY

SEQ ID NO: 37457 - protein, 9 aa, synthetic construct
GGRGADVAH

SEQ ID NO: 37458 - protein, 9 aa, synthetic construct
GGRGADSFC

SEQ ID NO: 37459 - protein, 9 aa, synthetic construct
GGRGADTIL

SEQ ID NO: 37460 - protein, 9 aa, synthetic construct
GGRGADSIA

SEQ ID NO: 37461 - protein, 9 aa, synthetic construct
GGRGADSIV

SEQ ID NO: 37462 - protein, 9 aa, synthetic construct
GGRGADSLH

SEQ ID NO: 37463 - protein, 9 aa, synthetic construct
GGRGADSLN

SEQ ID NO: 37464 - protein, 9 aa, synthetic construct
GGRGADSLV

SEQ ID NO: 37465 - protein, 9 aa, synthetic construct
GGRGADSMR

SEQ ID NO: 37466 - protein, 9 aa, synthetic construct
GGRGADTAL

SEQ ID NO: 37467 - protein, 9 aa, synthetic construct
GGRGADTFE

SEQ ID NO: 37468 - protein, 9 aa, synthetic construct
GGRGADTFF

SEQ ID NO: 37469 - protein, 9 aa, synthetic construct
GGRGADTFQ

SEQ ID NO: 37470 - protein, 9 aa, synthetic construct
GGRGADTFR

SEQ ID NO: 37471 - protein, 9 aa, synthetic construct
GGRGADTFY

SEQ ID NO: 37472 - protein, 9 aa, synthetic construct
GGRGADTIG

SEQ ID NO: 37473 - protein, 9 aa, synthetic construct
GGRGADTIQ

SEQ ID NO: 37474 - protein, 9 aa, synthetic construct
GGRGADTYR

SEQ ID NO: 37475 - protein, 9 aa, synthetic construct
GGRGADTIR

SEQ ID NO: 37476 - protein, 9 aa, synthetic construct
GGRGADTIT

SEQ ID NO: 37477 - protein, 9 aa, synthetic construct
GGRGADTIY

SEQ ID NO: 37478 - protein, 9 aa, synthetic construct
GGRGADTLA

SEQ ID NO: 37479 - protein, 9 aa, synthetic construct
GGRGADTLQ

SEQ ID NO: 37480 - protein, 9 aa, synthetic construct
GGRGADTLY

SEQ ID NO: 37481 - protein, 9 aa, synthetic construct
GGRGADTMF

SEQ ID NO: 37482 - protein, 9 aa, synthetic construct
GGRGADTML

SEQ ID NO: 37483 - protein, 9 aa, synthetic construct
GGRGADTMN

SEQ ID NO: 37484 - protein, 9 aa, synthetic construct
GGRGADTMY

SEQ ID NO: 37485 - protein, 9 aa, synthetic construct
GGRGADTVD

SEQ ID NO: 37486 - protein, 9 aa, synthetic construct
GGRGADTVY

SEQ ID NO: 37487 - protein, 9 aa, synthetic construct
GGRGADTYD

SEQ ID NO: 37488 - protein, 9 aa, synthetic construct
GGRGDDSMV

SEQ ID NO: 37489 - protein, 9 aa, synthetic construct
GGRGDDSYF

SEQ ID NO: 37490 - protein, 9 aa, synthetic construct
GGQGIDFAY

SEQ ID NO: 37491 - protein, 9 aa, synthetic construct
GGRGKDIIV

SEQ ID NO: 37492 - protein, 9 aa, synthetic construct
GGRGHDWIF

SEQ ID NO: 37493 - protein, 9 aa, synthetic construct
GGRGHDWLW

SEQ ID NO: 37494 - protein, 9 aa, synthetic construct
GGRGHDYVH

SEQ ID NO: 37495 - protein, 9 aa, synthetic construct
GGRGIDFVV

SEQ ID NO: 37496 - protein, 9 aa, synthetic construct
GGRGIDKMI

SEQ ID NO: 37497 - protein, 9 aa, synthetic construct
GGRGIDLLN

SEQ ID NO: 37498 - protein, 9 aa, synthetic construct
GGRGIDQMT

SEQ ID NO: 37499 - protein, 9 aa, synthetic construct
GGRGIDRIN

SEQ ID NO: 37500 - protein, 9 aa, synthetic construct
GGRGIDRLC

SEQ ID NO: 37501 - protein, 9 aa, synthetic construct
GGRGIDRMA

SEQ ID NO: 37502 - protein, 9 aa, synthetic construct
GGRGIDRME

SEQ ID NO: 37503 - protein, 9 aa, synthetic construct
GGRGIDRMK

SEQ ID NO: 37504 - protein, 9 aa, synthetic construct
GGRGIDSLD

SEQ ID NO: 37505 - protein, 9 aa, synthetic construct
GGRGIDSLM

SEQ ID NO: 37506 - protein, 9 aa, synthetic construct
GGRGIDTIR

SEQ ID NO: 37507 - protein, 9 aa, synthetic construct
GGRGIDTLF

SEQ ID NO: 37508 - protein, 9 aa, synthetic construct
GGRGIDTLK

SEQ ID NO: 37509 - protein, 9 aa, synthetic construct
GGRGIDTLT

SEQ ID NO: 37510 - protein, 9 aa, synthetic construct
GGRGIDTVR

SEQ ID NO: 37511 - protein, 9 aa, synthetic construct
GGRGIDVIF

SEQ ID NO: 37512 - protein, 9 aa, synthetic construct
GGRGIDVYI

SEQ ID NO: 37513 - protein, 9 aa, synthetic construct
GGRGIDWIN

SEQ ID NO: 37514 - protein, 9 aa, synthetic construct
GGRGIDWVN

SEQ ID NO: 37515 - protein, 9 aa, synthetic construct
GGRGKDDLR

SEQ ID NO: 37516 - protein, 9 aa, synthetic construct
GGRGKDDLS

SEQ ID NO: 37517 - protein, 9 aa, synthetic construct
GGRGKDFIY

SEQ ID NO: 37518 - protein, 9 aa, synthetic construct
GGRGKDFLD

SEQ ID NO: 37519 - protein, 9 aa, synthetic construct
GGRGKDFLS

SEQ ID NO: 37520 - protein, 9 aa, synthetic construct
GGRGKDGIF

SEQ ID NO: 37521 - protein, 9 aa, synthetic construct
GGRGHDVYV

SEQ ID NO: 37522 - protein, 9 aa, synthetic construct
GGRGHDVMT

SEQ ID NO: 37523 - protein, 9 aa, synthetic construct
GGRGHDVMR

SEQ ID NO: 37524 - protein, 9 aa, synthetic construct
GGRGHDQMS

SEQ ID NO: 37525 - protein, 9 aa, synthetic construct
GGRGHDIFV

SEQ ID NO: 37526 - protein, 9 aa, synthetic construct
GGRGHDIIA

SEQ ID NO: 37527 - protein, 9 aa, synthetic construct
GGRGHDILK

SEQ ID NO: 37528 - protein, 9 aa, synthetic construct
GGRGHDILN

SEQ ID NO: 37529 - protein, 9 aa, synthetic construct
GGRGHDKLY

SEQ ID NO: 37530 - protein, 9 aa, synthetic construct
GGRGHDLLE

SEQ ID NO: 37531 - protein, 9 aa, synthetic construct
GGRGHDLLR

SEQ ID NO: 37532 - protein, 9 aa, synthetic construct
GGRGHDLLT

SEQ ID NO: 37533 - protein, 9 aa, synthetic construct
GGRGHDLMG

SEQ ID NO: 37534 - protein, 9 aa, synthetic construct
GGRGHDMLS

SEQ ID NO: 37535 - protein, 9 aa, synthetic construct
GGRGHDNLF

SEQ ID NO: 37536 - protein, 9 aa, synthetic construct
GGRGHDNVV

SEQ ID NO: 37537 - protein, 9 aa, synthetic construct
GGRGHDQFF

SEQ ID NO: 37538 - protein, 9 aa, synthetic construct
GGRGHDRID

SEQ ID NO: 37539 - protein, 9 aa, synthetic construct
GGRGHDVLV

SEQ ID NO: 37540 - protein, 9 aa, synthetic construct
GGRGHDRLF

SEQ ID NO: 37541 - protein, 9 aa, synthetic construct
GGRGHDRLI

SEQ ID NO: 37542 - protein, 9 aa, synthetic construct
GGRGHDSIM

SEQ ID NO: 37543 - protein, 9 aa, synthetic construct
GGRGHDSLL

SEQ ID NO: 37544 - protein, 9 aa, synthetic construct
GGRGHDSMN

SEQ ID NO: 37545 - protein, 9 aa, synthetic construct
GGRGHDTIF

SEQ ID NO: 37546 - protein, 9 aa, synthetic construct
GGRGHDTIS

SEQ ID NO: 37547 - protein, 9 aa, synthetic construct
GGRGHDTLL

SEQ ID NO: 37548 - protein, 9 aa, synthetic construct
GGRGHDTLR

SEQ ID NO: 37549 - protein, 9 aa, synthetic construct
GGRGHDTLV

SEQ ID NO: 37550 - protein, 9 aa, synthetic construct
GGRGHDVIL

SEQ ID NO: 37551 - protein, 9 aa, synthetic construct
GGRGHDVLS

SEQ ID NO: 37552 - protein, 9 aa, synthetic construct
GGRGHDVLT

SEQ ID NO: 37553 - protein, 9 aa, synthetic construct
GGRGKDIFV

SEQ ID NO: 37554 - protein, 9 aa, synthetic construct
GGRGKDILI

SEQ ID NO: 37555 - protein, 9 aa, synthetic construct
GGRGDDTAW

SEQ ID NO: 37556 - protein, 9 aa, synthetic construct
GGRGKDILY

SEQ ID NO: 37557 - protein, 9 aa, synthetic construct
GGRGKDYLY

SEQ ID NO: 37558 - protein, 9 aa, synthetic construct
GGRGLDALF

SEQ ID NO: 37559 - protein, 9 aa, synthetic construct
GGRGLDILF

SEQ ID NO: 37560 - protein, 9 aa, synthetic construct
GGRGLDLID

SEQ ID NO: 37561 - protein, 9 aa, synthetic construct
GGRGLDLLD

SEQ ID NO: 37562 - protein, 9 aa, synthetic construct
GGRGLDLLM

SEQ ID NO: 37563 - protein, 9 aa, synthetic construct
GGRGLDLLY

SEQ ID NO: 37564 - protein, 9 aa, synthetic construct
GGRGLDMLS

SEQ ID NO: 37565 - protein, 9 aa, synthetic construct
GGRGLDNLD

SEQ ID NO: 37566 - protein, 9 aa, synthetic construct
GGRGLDRIF

SEQ ID NO: 37567 - protein, 9 aa, synthetic construct
GGRGLDRLD

SEQ ID NO: 37568 - protein, 9 aa, synthetic construct
GGRGLDRLE

SEQ ID NO: 37569 - protein, 9 aa, synthetic construct
GGRGLDRLN

SEQ ID NO: 37570 - protein, 9 aa, synthetic construct
GGRGLDRLT

SEQ ID NO: 37571 - protein, 9 aa, synthetic construct
GGRGLDRMF

SEQ ID NO: 37572 - protein, 9 aa, synthetic construct
GGRGLDTFV

SEQ ID NO: 37573 - protein, 9 aa, synthetic construct
GGRGLDTLT

SEQ ID NO: 37574 - protein, 9 aa, synthetic construct
GGRGLDVAG

SEQ ID NO: 37575 - protein, 9 aa, synthetic construct
GGRGLDVLD

SEQ ID NO: 37576 - protein, 9 aa, synthetic construct
GGRGLDVML

SEQ ID NO: 37577 - protein, 9 aa, synthetic construct
GGRGMDEII

SEQ ID NO: 37578 - protein, 9 aa, synthetic construct
GGRGMDELR

SEQ ID NO: 37579 - protein, 9 aa, synthetic construct
GGRGMDIMT

SEQ ID NO: 37580 - protein, 9 aa, synthetic construct
GGRGMDLLI

SEQ ID NO: 37581 - protein, 9 aa, synthetic construct
GGRGMDLLK

SEQ ID NO: 37582 - protein, 9 aa, synthetic construct
GGRGMDQVF

SEQ ID NO: 37583 - protein, 9 aa, synthetic construct
GGRGMDTIK

SEQ ID NO: 37584 - protein, 9 aa, synthetic construct
GGRGMDTIN

SEQ ID NO: 37585 - protein, 9 aa, synthetic construct
GGRGMDTLA

SEQ ID NO: 37586 - protein, 9 aa, synthetic construct
GGRGKDWLY

SEQ ID NO: 37587 - protein, 9 aa, synthetic construct
GGRGKDWLD

SEQ ID NO: 37588 - protein, 9 aa, synthetic construct
GGRGKDVMS

SEQ ID NO: 37589 - protein, 9 aa, synthetic construct
GGRGKDRID

SEQ ID NO: 37590 - protein, 9 aa, synthetic construct
GGRGKDIYY

SEQ ID NO: 37591 - protein, 9 aa, synthetic construct
GGRGKDKIL

SEQ ID NO: 37592 - protein, 9 aa, synthetic construct
GGRGKDKLA

SEQ ID NO: 37593 - protein, 9 aa, synthetic construct
GGRGKDKLY

SEQ ID NO: 37594 - protein, 9 aa, synthetic construct
GGRGKDLFL

SEQ ID NO: 37595 - protein, 9 aa, synthetic construct
GGRGKDLLN

SEQ ID NO: 37596 - protein, 9 aa, synthetic construct
GGRGKDLLQ

SEQ ID NO: 37597 - protein, 9 aa, synthetic construct
GGRGKDLLV

SEQ ID NO: 37598 - protein, 9 aa, synthetic construct
GGRGKDLMD

SEQ ID NO: 37599 - protein, 9 aa, synthetic construct
GGRGKDMLT

SEQ ID NO: 37600 - protein, 9 aa, synthetic construct
GGRGKDNLN

SEQ ID NO: 37601 - protein, 9 aa, synthetic construct
GGRGKDQFV

SEQ ID NO: 37602 - protein, 9 aa, synthetic construct
GGRGKDQLS

SEQ ID NO: 37603 - protein, 9 aa, synthetic construct
GGRGKDRIE

SEQ ID NO: 37604 - protein, 9 aa, synthetic construct
GGRGKDVMF

SEQ ID NO: 37605 - protein, 9 aa, synthetic construct
GGRGKDRIK

SEQ ID NO: 37606 - protein, 9 aa, synthetic construct
GGRGKDRLI

SEQ ID NO: 37607 - protein, 9 aa, synthetic construct
GGRGKDRMS

SEQ ID NO: 37608 - protein, 9 aa, synthetic construct
GGRGKDRMT

SEQ ID NO: 37609 - protein, 9 aa, synthetic construct
GGRGKDSLW

SEQ ID NO: 37610 - protein, 9 aa, synthetic construct
GGRGKDSLY

SEQ ID NO: 37611 - protein, 9 aa, synthetic construct
GGRGKDTAI

SEQ ID NO: 37612 - protein, 9 aa, synthetic construct
GGRGKDTFI

SEQ ID NO: 37613 - protein, 9 aa, synthetic construct
GGRGKDTFV

SEQ ID NO: 37614 - protein, 9 aa, synthetic construct
GGRGKDTLE

SEQ ID NO: 37615 - protein, 9 aa, synthetic construct
GGRGKDTLN

SEQ ID NO: 37616 - protein, 9 aa, synthetic construct
GGRGKDVLL

SEQ ID NO: 37617 - protein, 9 aa, synthetic construct
GGRGKDVLW

SEQ ID NO: 37618 - protein, 9 aa, synthetic construct
GGRGHDHIT

SEQ ID NO: 37619 - protein, 9 aa, synthetic construct
GGRGHDGID

SEQ ID NO: 37620 - protein, 9 aa, synthetic construct
GGRGHDFMR

SEQ ID NO: 37621 - protein, 9 aa, synthetic construct
GGRGHDFLY

SEQ ID NO: 37622 - protein, 9 aa, synthetic construct
GGRGDDYLK

SEQ ID NO: 37623 - protein, 9 aa, synthetic construct
GGRGDDYLV

SEQ ID NO: 37624 - protein, 9 aa, synthetic construct
GGRGDDYLY

SEQ ID NO: 37625 - protein, 9 aa, synthetic construct
GGRGDDYME

SEQ ID NO: 37626 - protein, 9 aa, synthetic construct
GGRGDDYML

SEQ ID NO: 37627 - protein, 9 aa, synthetic construct
GGRGDDYYI

SEQ ID NO: 37628 - protein, 9 aa, synthetic construct
GGRGDDYYS

SEQ ID NO: 37629 - protein, 9 aa, synthetic construct
GGRGEDDIS

SEQ ID NO: 37630 - protein, 9 aa, synthetic construct
GGRGEDDLE

SEQ ID NO: 37631 - protein, 9 aa, synthetic construct
GGRGEDELH

SEQ ID NO: 37632 - protein, 9 aa, synthetic construct
GGRGEDELM

SEQ ID NO: 37633 - protein, 9 aa, synthetic construct
GGRGEDFIE

SEQ ID NO: 37634 - protein, 9 aa, synthetic construct
GGRGEDFLD

SEQ ID NO: 37635 - protein, 9 aa, synthetic construct
GGRGEDHLG

SEQ ID NO: 37636 - protein, 9 aa, synthetic construct
GGRGEDHVL

SEQ ID NO: 37637 - protein, 9 aa, synthetic construct
GGRGEDKLF

SEQ ID NO: 37638 - protein, 9 aa, synthetic construct
GGRGEDLLK

SEQ ID NO: 37639 - protein, 9 aa, synthetic construct
GGRGEDLLT

SEQ ID NO: 37640 - protein, 9 aa, synthetic construct
GGRGEDMIH

SEQ ID NO: 37641 - protein, 9 aa, synthetic construct
GGRGEDNLH

SEQ ID NO: 37642 - protein, 9 aa, synthetic construct
GGRGEDRLA

SEQ ID NO: 37643 - protein, 9 aa, synthetic construct
GGRGEDRLD

SEQ ID NO: 37644 - protein, 9 aa, synthetic construct
GGRGEDRLT

SEQ ID NO: 37645 - protein, 9 aa, synthetic construct
GGRGEDRLV

SEQ ID NO: 37646 - protein, 9 aa, synthetic construct
GGRGEDSIN

SEQ ID NO: 37647 - protein, 9 aa, synthetic construct
GGRGEDTID

SEQ ID NO: 37648 - protein, 9 aa, synthetic construct
GGRGEDTII

SEQ ID NO: 37649 - protein, 9 aa, synthetic construct
GGRGEDTIR

SEQ ID NO: 37650 - protein, 9 aa, synthetic construct
GGRGEDTLA

SEQ ID NO: 37651 - protein, 9 aa, synthetic construct
GGRGDDYLI

SEQ ID NO: 37652 - protein, 9 aa, synthetic construct
GGRGDDWMT

SEQ ID NO: 37653 - protein, 9 aa, synthetic construct
GGRGDDWLR

SEQ ID NO: 37654 - protein, 9 aa, synthetic construct
GGRGDDVAQ

SEQ ID NO: 37655 - protein, 9 aa, synthetic construct
GGRGDDTIF

SEQ ID NO: 37656 - protein, 9 aa, synthetic construct
GGRGDDTIH

SEQ ID NO: 37657 - protein, 9 aa, synthetic construct
GGRGDDTIV

SEQ ID NO: 37658 - protein, 9 aa, synthetic construct
GGRGDDTLW

SEQ ID NO: 37659 - protein, 9 aa, synthetic construct
GGRGDDTMH

SEQ ID NO: 37660 - protein, 9 aa, synthetic construct
GGRGDDTMV

SEQ ID NO: 37661 - protein, 9 aa, synthetic construct
GGRGDDTMY

SEQ ID NO: 37662 - protein, 9 aa, synthetic construct
GGRGDDTVE

SEQ ID NO: 37663 - protein, 9 aa, synthetic construct
GGRGDDTVI

SEQ ID NO: 37664 - protein, 9 aa, synthetic construct
GGRGDDTVK

SEQ ID NO: 37665 - protein, 9 aa, synthetic construct
GGRGDDTVV

SEQ ID NO: 37666 - protein, 9 aa, synthetic construct
GGRGDDTVW

SEQ ID NO: 37667 - protein, 9 aa, synthetic construct
GGRGDDTYD

SEQ ID NO: 37668 - protein, 9 aa, synthetic construct
GGRGDDVIF

SEQ ID NO: 37669 - protein, 9 aa, synthetic construct
GGRGDDWLI

SEQ ID NO: 37670 - protein, 9 aa, synthetic construct
GGRGDDVIN

SEQ ID NO: 37671 - protein, 9 aa, synthetic construct
GGRGDDVLM

SEQ ID NO: 37672 - protein, 9 aa, synthetic construct
GGRGDDVME

SEQ ID NO: 37673 - protein, 9 aa, synthetic construct
GGRGDDVMG

SEQ ID NO: 37674 - protein, 9 aa, synthetic construct
GGRGDDVMR

SEQ ID NO: 37675 - protein, 9 aa, synthetic construct
GGRGDDVMS

SEQ ID NO: 37676 - protein, 9 aa, synthetic construct
GGRGDDVVK

SEQ ID NO: 37677 - protein, 9 aa, synthetic construct
GGRGDDVVL

SEQ ID NO: 37678 - protein, 9 aa, synthetic construct
GGRGDDVVR

SEQ ID NO: 37679 - protein, 9 aa, synthetic construct
GGRGDDVYL

SEQ ID NO: 37680 - protein, 9 aa, synthetic construct
GGRGDDVYT

SEQ ID NO: 37681 - protein, 9 aa, synthetic construct
GGRGDDWID

SEQ ID NO: 37682 - protein, 9 aa, synthetic construct
GGRGDDWLF

SEQ ID NO: 37683 - protein, 9 aa, synthetic construct
GGRGEDTLL

SEQ ID NO: 37684 - protein, 9 aa, synthetic construct
GGRGEDTLM

SEQ ID NO: 37685 - protein, 9 aa, synthetic construct
GGRGEDTLN

SEQ ID NO: 37686 - protein, 9 aa, synthetic construct
GGRGGDTFF

SEQ ID NO: 37687 - protein, 9 aa, synthetic construct
GGRGGDLLV

SEQ ID NO: 37688 - protein, 9 aa, synthetic construct
GGRGGDLVL

SEQ ID NO: 37689 - protein, 9 aa, synthetic construct
GGRGGDMLQ

SEQ ID NO: 37690 - protein, 9 aa, synthetic construct
GGRGGDMVA

SEQ ID NO: 37691 - protein, 9 aa, synthetic construct
GGRGGDMVN

SEQ ID NO: 37692 - protein, 9 aa, synthetic construct
GGRGGDRAI

SEQ ID NO: 37693 - protein, 9 aa, synthetic construct
GGRGGDRLE

SEQ ID NO: 37694 - protein, 9 aa, synthetic construct
GGRGGDRMA

SEQ ID NO: 37695 - protein, 9 aa, synthetic construct
GGRGGDRMK

SEQ ID NO: 37696 - protein, 9 aa, synthetic construct
GGRGGDSLA

SEQ ID NO: 37697 - protein, 9 aa, synthetic construct
GGRGGDSLF

SEQ ID NO: 37698 - protein, 9 aa, synthetic construct
GGRGGDSMR

SEQ ID NO: 37699 - protein, 9 aa, synthetic construct
GGRGGDTAV

SEQ ID NO: 37700 - protein, 9 aa, synthetic construct
GGRGGDTIM

SEQ ID NO: 37701 - protein, 9 aa, synthetic construct
GGRGGDLLN

SEQ ID NO: 37702 - protein, 9 aa, synthetic construct
GGRGGDTIN

SEQ ID NO: 37703 - protein, 9 aa, synthetic construct
GGRGGDTIS

SEQ ID NO: 37704 - protein, 9 aa, synthetic construct
GGRGGDTLS

SEQ ID NO: 37705 - protein, 9 aa, synthetic construct
GGRGGDTLW

SEQ ID NO: 37706 - protein, 9 aa, synthetic construct
GGRGGDVFI

SEQ ID NO: 37707 - protein, 9 aa, synthetic construct
GGRGGDVIF

SEQ ID NO: 37708 - protein, 9 aa, synthetic construct
GGRGGDVIS

SEQ ID NO: 37709 - protein, 9 aa, synthetic construct
GGRGGDVLS

SEQ ID NO: 37710 - protein, 9 aa, synthetic construct
GGRGGDVMV

SEQ ID NO: 37711 - protein, 9 aa, synthetic construct
GGRGGDWLD

SEQ ID NO: 37712 - protein, 9 aa, synthetic construct
GGRGHDEIE

SEQ ID NO: 37713 - protein, 9 aa, synthetic construct
GGRGHDELQ

SEQ ID NO: 37714 - protein, 9 aa, synthetic construct
GGRGHDFIF

SEQ ID NO: 37715 - protein, 9 aa, synthetic construct
GGRGGDLLT

SEQ ID NO: 37716 - protein, 9 aa, synthetic construct
GGRGGDLLF

SEQ ID NO: 37717 - protein, 9 aa, synthetic construct
GGRGEDTLT

SEQ ID NO: 37718 - protein, 9 aa, synthetic construct
GGRGFDLLD

SEQ ID NO: 37719 - protein, 9 aa, synthetic construct
GGRGEDTMT

SEQ ID NO: 37720 - protein, 9 aa, synthetic construct
GGRGEDTVR

SEQ ID NO: 37721 - protein, 9 aa, synthetic construct
GGRGEDTYV

SEQ ID NO: 37722 - protein, 9 aa, synthetic construct
GGRGEDVIE

SEQ ID NO: 37723 - protein, 9 aa, synthetic construct
GGRGEDVLF

SEQ ID NO: 37724 - protein, 9 aa, synthetic construct
GGRGEDVLS

SEQ ID NO: 37725 - protein, 9 aa, synthetic construct
GGRGEDYLS

SEQ ID NO: 37726 - protein, 9 aa, synthetic construct
GGRGEDYVD

SEQ ID NO: 37727 - protein, 9 aa, synthetic construct
GGRGFDAVD

SEQ ID NO: 37728 - protein, 9 aa, synthetic construct
GGRGFDDLN

SEQ ID NO: 37729 - protein, 9 aa, synthetic construct
GGRGFDEIS

SEQ ID NO: 37730 - protein, 9 aa, synthetic construct
GGRGFDEMY

SEQ ID NO: 37731 - protein, 9 aa, synthetic construct
GGRGFDFID

SEQ ID NO: 37732 - protein, 9 aa, synthetic construct
GGRGFDQID

SEQ ID NO: 37733 - protein, 9 aa, synthetic construct
GGRGGDKLY

SEQ ID NO: 37734 - protein, 9 aa, synthetic construct
GGRGFDRLS

SEQ ID NO: 37735 - protein, 9 aa, synthetic construct
GGRGFDRLY

SEQ ID NO: 37736 - protein, 9 aa, synthetic construct
GGRGFDRVI

SEQ ID NO: 37737 - protein, 9 aa, synthetic construct
GGRGFDSLD

SEQ ID NO: 37738 - protein, 9 aa, synthetic construct
GGRGFDVFV

SEQ ID NO: 37739 - protein, 9 aa, synthetic construct
GGRGFDWAT

SEQ ID NO: 37740 - protein, 9 aa, synthetic construct
GGRGFDYAD

SEQ ID NO: 37741 - protein, 9 aa, synthetic construct
GGRGGDALE

SEQ ID NO: 37742 - protein, 9 aa, synthetic construct
GGRGGDEIW

SEQ ID NO: 37743 - protein, 9 aa, synthetic construct
GGRGGDELD

SEQ ID NO: 37744 - protein, 9 aa, synthetic construct
GGRGGDEYY

SEQ ID NO: 37745 - protein, 9 aa, synthetic construct
GGRGGDGLQ

SEQ ID NO: 37746 - protein, 9 aa, synthetic construct
GGRGGDHLW

SEQ ID NO: 37747 - protein, 9 aa, synthetic construct
GGQGYDYIF

SEQ ID NO: 37748 - protein, 9 aa, synthetic construct
GGQGYDTLD

SEQ ID NO: 37749 - protein, 9 aa, synthetic construct
GGQGYDSYV

SEQ ID NO: 37750 - protein, 9 aa, synthetic construct
GGQGNDSVA

SEQ ID NO: 37751 - protein, 9 aa, synthetic construct
GGQGNDNVR

SEQ ID NO: 37752 - protein, 9 aa, synthetic construct
GGQGNDNYL

SEQ ID NO: 37753 - protein, 9 aa, synthetic construct
GGQGNDPLV

SEQ ID NO: 37754 - protein, 9 aa, synthetic construct
GGQGNDQID

SEQ ID NO: 37755 - protein, 9 aa, synthetic construct
GGQGNDQIN

SEQ ID NO: 37756 - protein, 9 aa, synthetic construct
GGQGNDQIQ

SEQ ID NO: 37757 - protein, 9 aa, synthetic construct
GGQGNDQIS

SEQ ID NO: 37758 - protein, 9 aa, synthetic construct
GGQGNDQLA

SEQ ID NO: 37759 - protein, 9 aa, synthetic construct
GGQGNDQLL

SEQ ID NO: 37760 - protein, 9 aa, synthetic construct
GGQGNDQLW

SEQ ID NO: 37761 - protein, 9 aa, synthetic construct
GGQGNDQMF

SEQ ID NO: 37762 - protein, 9 aa, synthetic construct
GGQGNDQVY

SEQ ID NO: 37763 - protein, 9 aa, synthetic construct
GGQGNDRFE

SEQ ID NO: 37764 - protein, 9 aa, synthetic construct
GGQGNDRID

SEQ ID NO: 37765 - protein, 9 aa, synthetic construct
GGQGNDRIF

SEQ ID NO: 37766 - protein, 9 aa, synthetic construct
GGQGNDRLA

SEQ ID NO: 37767 - protein, 9 aa, synthetic construct
GGQGNDRLN

SEQ ID NO: 37768 - protein, 9 aa, synthetic construct
GGQGNDRLR

SEQ ID NO: 37769 - protein, 9 aa, synthetic construct
GGQGNDRMF

SEQ ID NO: 37770 - protein, 9 aa, synthetic construct
GGQGNDRVF

SEQ ID NO: 37771 - protein, 9 aa, synthetic construct
GGQGNDRVY

SEQ ID NO: 37772 - protein, 9 aa, synthetic construct
GGQGNDSIE

SEQ ID NO: 37773 - protein, 9 aa, synthetic construct
GGQGNDSIP

SEQ ID NO: 37774 - protein, 9 aa, synthetic construct
GGQGNDSIT

SEQ ID NO: 37775 - protein, 9 aa, synthetic construct
GGQGNDSIY

SEQ ID NO: 37776 - protein, 9 aa, synthetic construct
GGQGNDSLE

SEQ ID NO: 37777 - protein, 9 aa, synthetic construct
GGQGNDSLG

SEQ ID NO: 37778 - protein, 9 aa, synthetic construct
GGQGNDSMD

SEQ ID NO: 37779 - protein, 9 aa, synthetic construct
GGQGNDSMF

SEQ ID NO: 37780 - protein, 9 aa, synthetic construct
GGQGNDNLY

SEQ ID NO: 37781 - protein, 9 aa, synthetic construct
GGQGNDNLR

SEQ ID NO: 37782 - protein, 9 aa, synthetic construct
GGQGNDNLN

SEQ ID NO: 37783 - protein, 9 aa, synthetic construct
GGQGNDLLG

SEQ ID NO: 37784 - protein, 9 aa, synthetic construct
GGQGNDILK

SEQ ID NO: 37785 - protein, 9 aa, synthetic construct
GGQGNDIVH

SEQ ID NO: 37786 - protein, 9 aa, synthetic construct
GGQGNDIVQ

SEQ ID NO: 37787 - protein, 9 aa, synthetic construct
GGQGNDKFD

SEQ ID NO: 37788 - protein, 9 aa, synthetic construct
GGQGNDKIN

SEQ ID NO: 37789 - protein, 9 aa, synthetic construct
GGQGNDKLG

SEQ ID NO: 37790 - protein, 9 aa, synthetic construct
GGQGNDKLQ

SEQ ID NO: 37791 - protein, 9 aa, synthetic construct
GGQGNDLAF

SEQ ID NO: 37792 - protein, 9 aa, synthetic construct
GGQGNDLFQ

SEQ ID NO: 37793 - protein, 9 aa, synthetic construct
GGQGNDLIE

SEQ ID NO: 37794 - protein, 9 aa, synthetic construct
GGQGNDLIF

SEQ ID NO: 37795 - protein, 9 aa, synthetic construct
GGQGNDLIK

SEQ ID NO: 37796 - protein, 9 aa, synthetic construct
GGQGNDLIN

SEQ ID NO: 37797 - protein, 9 aa, synthetic construct
GGQGNDLML

SEQ ID NO: 37798 - protein, 9 aa, synthetic construct
GGQGNDNLL

SEQ ID NO: 37799 - protein, 9 aa, synthetic construct
GGQGNDLVC

SEQ ID NO: 37800 - protein, 9 aa, synthetic construct
GGQGNDLVH

SEQ ID NO: 37801 - protein, 9 aa, synthetic construct
GGQGNDLVL

SEQ ID NO: 37802 - protein, 9 aa, synthetic construct
GGQGNDLVS

SEQ ID NO: 37803 - protein, 9 aa, synthetic construct
GGQGNDLYG

SEQ ID NO: 37804 - protein, 9 aa, synthetic construct
GGQGNDMAV

SEQ ID NO: 37805 - protein, 9 aa, synthetic construct
GGQGNDMLD

SEQ ID NO: 37806 - protein, 9 aa, synthetic construct
GGQGNDMLN

SEQ ID NO: 37807 - protein, 9 aa, synthetic construct
GGQGNDMVL

SEQ ID NO: 37808 - protein, 9 aa, synthetic construct
GGQGNDNII

SEQ ID NO: 37809 - protein, 9 aa, synthetic construct
GGQGNDNIL

SEQ ID NO: 37810 - protein, 9 aa, synthetic construct
GGQGNDNIQ

SEQ ID NO: 37811 - protein, 9 aa, synthetic construct
GGQGNDNIR

SEQ ID NO: 37812 - protein, 9 aa, synthetic construct
GGQGNDSMN

SEQ ID NO: 37813 - protein, 9 aa, synthetic construct
GGQGNDSVF

SEQ ID NO: 37814 - protein, 9 aa, synthetic construct
GGQGYDSYA

SEQ ID NO: 37815 - protein, 9 aa, synthetic construct
GGQGNDSVG

SEQ ID NO: 37816 - protein, 9 aa, synthetic construct
GGQGNDVMV

SEQ ID NO: 37817 - protein, 9 aa, synthetic construct
GGQGNDVVE

SEQ ID NO: 37818 - protein, 9 aa, synthetic construct
GGQGNDVVG

SEQ ID NO: 37819 - protein, 9 aa, synthetic construct
GGQGNDVVN

SEQ ID NO: 37820 - protein, 9 aa, synthetic construct
GGQGNDVVR

SEQ ID NO: 37821 - protein, 9 aa, synthetic construct
GGQGNDVVS

SEQ ID NO: 37822 - protein, 9 aa, synthetic construct
GGQGNDVVY

SEQ ID NO: 37823 - protein, 9 aa, synthetic construct
GGQGNDVYI

SEQ ID NO: 37824 - protein, 9 aa, synthetic construct
GGQGNDWID

SEQ ID NO: 37825 - protein, 9 aa, synthetic construct
GGQGNDWLT

SEQ ID NO: 37826 - protein, 9 aa, synthetic construct
GGQGNDWLV

SEQ ID NO: 37827 - protein, 9 aa, synthetic construct
GGQGNDWVF

SEQ ID NO: 37828 - protein, 9 aa, synthetic construct
GGQGNDXLL

SEQ ID NO: 37829 - protein, 9 aa, synthetic construct
GGQGNDYIF

SEQ ID NO: 37830 - protein, 9 aa, synthetic construct
GGQGNDYIH

SEQ ID NO: 37831 - protein, 9 aa, synthetic construct
GGQGNDYIT

SEQ ID NO: 37832 - protein, 9 aa, synthetic construct
GGQGNDYLA

SEQ ID NO: 37833 - protein, 9 aa, synthetic construct
GGQGNDYLF

SEQ ID NO: 37834 - protein, 9 aa, synthetic construct
GGQGNDYLI

SEQ ID NO: 37835 - protein, 9 aa, synthetic construct
GGQGNDYLR

SEQ ID NO: 37836 - protein, 9 aa, synthetic construct
GGQGNDYLS

SEQ ID NO: 37837 - protein, 9 aa, synthetic construct
GGQGNDYVE

SEQ ID NO: 37838 - protein, 9 aa, synthetic construct
GGQGNDYVL

SEQ ID NO: 37839 - protein, 9 aa, synthetic construct
GGQGPDNLS

SEQ ID NO: 37840 - protein, 9 aa, synthetic construct
GGQGPDRLA

SEQ ID NO: 37841 - protein, 9 aa, synthetic construct
GGQGPDTLN

SEQ ID NO: 37842 - protein, 9 aa, synthetic construct
GGQGPDTLV

SEQ ID NO: 37843 - protein, 9 aa, synthetic construct
GGQGQDALR

SEQ ID NO: 37844 - protein, 9 aa, synthetic construct
GGQGQDALS

SEQ ID NO: 37845 - protein, 9 aa, synthetic construct
GGQGNDVMS

SEQ ID NO: 37846 - protein, 9 aa, synthetic construct
GGQGNDVMQ

SEQ ID NO: 37847 - protein, 9 aa, synthetic construct
GGQGNDVLF

SEQ ID NO: 37848 - protein, 9 aa, synthetic construct
GGQGNDTMD

SEQ ID NO: 37849 - protein, 9 aa, synthetic construct
GGQGNDSVL

SEQ ID NO: 37850 - protein, 9 aa, synthetic construct
GGQGNDSVN

SEQ ID NO: 37851 - protein, 9 aa, synthetic construct
GGQGNDSVQ

SEQ ID NO: 37852 - protein, 9 aa, synthetic construct
GGQGNDSVY

SEQ ID NO: 37853 - protein, 9 aa, synthetic construct
GGQGNDSYF

SEQ ID NO: 37854 - protein, 9 aa, synthetic construct
GGQGNDSYY

SEQ ID NO: 37855 - protein, 9 aa, synthetic construct
GGQGNDTAI

SEQ ID NO: 37856 - protein, 9 aa, synthetic construct
GGQGNDTIA

SEQ ID NO: 37857 - protein, 9 aa, synthetic construct
GGQGNDTIG

SEQ ID NO: 37858 - protein, 9 aa, synthetic construct
GGQGNDTII

SEQ ID NO: 37859 - protein, 9 aa, synthetic construct
GGQGNDTIM

SEQ ID NO: 37860 - protein, 9 aa, synthetic construct
GGQGNDTIW

SEQ ID NO: 37861 - protein, 9 aa, synthetic construct
GGQGNDTLC

SEQ ID NO: 37862 - protein, 9 aa, synthetic construct
GGQGNDTMG

SEQ ID NO: 37863 - protein, 9 aa, synthetic construct
GGQGNDVLE

SEQ ID NO: 37864 - protein, 9 aa, synthetic construct
GGQGNDTMR

SEQ ID NO: 37865 - protein, 9 aa, synthetic construct
GGQGNDTMV

SEQ ID NO: 37866 - protein, 9 aa, synthetic construct
GGQGNDTVN

SEQ ID NO: 37867 - protein, 9 aa, synthetic construct
GGQGNDTVT

SEQ ID NO: 37868 - protein, 9 aa, synthetic construct
GGQGNDTVV

SEQ ID NO: 37869 - protein, 9 aa, synthetic construct
GGQGNDTYF

SEQ ID NO: 37870 - protein, 9 aa, synthetic construct
GGQGNDTYK

SEQ ID NO: 37871 - protein, 9 aa, synthetic construct
GGQGNDTYN

SEQ ID NO: 37872 - protein, 9 aa, synthetic construct
GGQGNDVAV

SEQ ID NO: 37873 - protein, 9 aa, synthetic construct
GGQGNDVFR

SEQ ID NO: 37874 - protein, 9 aa, synthetic construct
GGQGNDVFT

SEQ ID NO: 37875 - protein, 9 aa, synthetic construct
GGQGNDVIG

SEQ ID NO: 37876 - protein, 9 aa, synthetic construct
GGQGNDVIR

SEQ ID NO: 37877 - protein, 9 aa, synthetic construct
GGQGNDILH

SEQ ID NO: 37878 - protein, 9 aa, synthetic construct
GGQGNDILG

SEQ ID NO: 37879 - protein, 9 aa, synthetic construct
GGQGNDILE

SEQ ID NO: 37880 - protein, 9 aa, synthetic construct
GGQGNDIIS

SEQ ID NO: 37881 - protein, 9 aa, synthetic construct
GGQGKDRLS

SEQ ID NO: 37882 - protein, 9 aa, synthetic construct
GGQGKDSFV

SEQ ID NO: 37883 - protein, 9 aa, synthetic construct
GGQGKDSYD

SEQ ID NO: 37884 - protein, 9 aa, synthetic construct
GGQGKDTLD

SEQ ID NO: 37885 - protein, 9 aa, synthetic construct
GGQGKDTLF

SEQ ID NO: 37886 - protein, 9 aa, synthetic construct
GGQGKDTLH

SEQ ID NO: 37887 - protein, 9 aa, synthetic construct
GGQGKDTLL

SEQ ID NO: 37888 - protein, 9 aa, synthetic construct
GGQGKDTLS

SEQ ID NO: 37889 - protein, 9 aa, synthetic construct
GGQGKDTLT

SEQ ID NO: 37890 - protein, 9 aa, synthetic construct
GGQGKDTLV

SEQ ID NO: 37891 - protein, 9 aa, synthetic construct
GGQGKDVFR

SEQ ID NO: 37892 - protein, 9 aa, synthetic construct
GGQGKDVLD

SEQ ID NO: 37893 - protein, 9 aa, synthetic construct
GGQGKDYFY

SEQ ID NO: 37894 - protein, 9 aa, synthetic construct
GGQGKDYLT

SEQ ID NO: 37895 - protein, 9 aa, synthetic construct
GGQGLDAMH

SEQ ID NO: 37896 - protein, 9 aa, synthetic construct
GGQGLDFLT

SEQ ID NO: 37897 - protein, 9 aa, synthetic construct
GGQGLDILT

SEQ ID NO: 37898 - protein, 9 aa, synthetic construct
GGQGLDILV

SEQ ID NO: 37899 - protein, 9 aa, synthetic construct
GGQGLDILW

SEQ ID NO: 37900 - protein, 9 aa, synthetic construct
GGQGLDKLD

SEQ ID NO: 37901 - protein, 9 aa, synthetic construct
GGQGLDMMY

SEQ ID NO: 37902 - protein, 9 aa, synthetic construct
GGQGLDNLY

SEQ ID NO: 37903 - protein, 9 aa, synthetic construct
GGQGLDNVY

SEQ ID NO: 37904 - protein, 9 aa, synthetic construct
GGQGLDQFV

SEQ ID NO: 37905 - protein, 9 aa, synthetic construct
GGQGLDRIE

SEQ ID NO: 37906 - protein, 9 aa, synthetic construct
GGQGLDRLT

SEQ ID NO: 37907 - protein, 9 aa, synthetic construct
GGQGLDSIL

SEQ ID NO: 37908 - protein, 9 aa, synthetic construct
GGQGLDSLT

SEQ ID NO: 37909 - protein, 9 aa, synthetic construct
GGQGLDTAV

SEQ ID NO: 37910 - protein, 9 aa, synthetic construct
GGQGKDRLE

SEQ ID NO: 37911 - protein, 9 aa, synthetic construct
GGQGKDQLE

SEQ ID NO: 37912 - protein, 9 aa, synthetic construct
GGQGKDLLL

SEQ ID NO: 37913 - protein, 9 aa, synthetic construct
GGQGIDVLN

SEQ ID NO: 37914 - protein, 9 aa, synthetic construct
GGQGIDFMD

SEQ ID NO: 37915 - protein, 9 aa, synthetic construct
GGQGIDHLD

SEQ ID NO: 37916 - protein, 9 aa, synthetic construct
GGQGIDIAS

SEQ ID NO: 37917 - protein, 9 aa, synthetic construct
GGQGIDILV

SEQ ID NO: 37918 - protein, 9 aa, synthetic construct
GGQGIDLMF

SEQ ID NO: 37919 - protein, 9 aa, synthetic construct
GGQGIDMLI

SEQ ID NO: 37920 - protein, 9 aa, synthetic construct
GGQGIDQFV

SEQ ID NO: 37921 - protein, 9 aa, synthetic construct
GGQGIDQLT

SEQ ID NO: 37922 - protein, 9 aa, synthetic construct
GGQGIDTAT

SEQ ID NO: 37923 - protein, 9 aa, synthetic construct
GGQGIDTAV

SEQ ID NO: 37924 - protein, 9 aa, synthetic construct
GGQGIDTLY

SEQ ID NO: 37925 - protein, 9 aa, synthetic construct
GGQGIDTMT

SEQ ID NO: 37926 - protein, 9 aa, synthetic construct
GGQGIDTVY

SEQ ID NO: 37927 - protein, 9 aa, synthetic construct
GGQGIDWAS

SEQ ID NO: 37928 - protein, 9 aa, synthetic construct
GGQGKDLIY

SEQ ID NO: 37929 - protein, 9 aa, synthetic construct
GGQGIDYLV

SEQ ID NO: 37930 - protein, 9 aa, synthetic construct
GGQGKDALY

SEQ ID NO: 37931 - protein, 9 aa, synthetic construct
GGQGKDAVY

SEQ ID NO: 37932 - protein, 9 aa, synthetic construct
GGQGKDDIT

SEQ ID NO: 37933 - protein, 9 aa, synthetic construct
GGQGKDEFH

SEQ ID NO: 37934 - protein, 9 aa, synthetic construct
GGQGKDFLA

SEQ ID NO: 37935 - protein, 9 aa, synthetic construct
GGQGKDFLS

SEQ ID NO: 37936 - protein, 9 aa, synthetic construct
GGQGKDFVD

SEQ ID NO: 37937 - protein, 9 aa, synthetic construct
GGQGKDILD

SEQ ID NO: 37938 - protein, 9 aa, synthetic construct
GGQGKDILE

SEQ ID NO: 37939 - protein, 9 aa, synthetic construct
GGQGKDILI

SEQ ID NO: 37940 - protein, 9 aa, synthetic construct
GGQGKDKLF

SEQ ID NO: 37941 - protein, 9 aa, synthetic construct
GGQGKDLIN

SEQ ID NO: 37942 - protein, 9 aa, synthetic construct
GGQGLDTLH

SEQ ID NO: 37943 - protein, 9 aa, synthetic construct
GGQGLDTLI

SEQ ID NO: 37944 - protein, 9 aa, synthetic construct
GGQGLDTLV

SEQ ID NO: 37945 - protein, 9 aa, synthetic construct
GGQGNDFML

SEQ ID NO: 37946 - protein, 9 aa, synthetic construct
GGQGNDEFT

SEQ ID NO: 37947 - protein, 9 aa, synthetic construct
GGQGNDEIA

SEQ ID NO: 37948 - protein, 9 aa, synthetic construct
GGQGNDEIE

SEQ ID NO: 37949 - protein, 9 aa, synthetic construct
GGQGNDEIF

SEQ ID NO: 37950 - protein, 9 aa, synthetic construct
GGQGNDELN

SEQ ID NO: 37951 - protein, 9 aa, synthetic construct
GGQGNDELQ

SEQ ID NO: 37952 - protein, 9 aa, synthetic construct
GGQGNDELT

SEQ ID NO: 37953 - protein, 9 aa, synthetic construct
GGQGNDELY

SEQ ID NO: 37954 - protein, 9 aa, synthetic construct
GGQGNDFFY

SEQ ID NO: 37955 - protein, 9 aa, synthetic construct
GGQGNDFLH

SEQ ID NO: 37956 - protein, 9 aa, synthetic construct
GGQGNDFLT

SEQ ID NO: 37957 - protein, 9 aa, synthetic construct
GGQGNDFLV

SEQ ID NO: 37958 - protein, 9 aa, synthetic construct
GGQGNDFMH

SEQ ID NO: 37959 - protein, 9 aa, synthetic construct
GGQGNDFVF

SEQ ID NO: 37960 - protein, 9 aa, synthetic construct
GGQGNDDLY

SEQ ID NO: 37961 - protein, 9 aa, synthetic construct
GGQGNDGIA

SEQ ID NO: 37962 - protein, 9 aa, synthetic construct
GGQGNDGLM

SEQ ID NO: 37963 - protein, 9 aa, synthetic construct
GGQGNDHAW

SEQ ID NO: 37964 - protein, 9 aa, synthetic construct
GGQGNDHII

SEQ ID NO: 37965 - protein, 9 aa, synthetic construct
GGQGNDHIS

SEQ ID NO: 37966 - protein, 9 aa, synthetic construct
GGQGNDHLY

SEQ ID NO: 37967 - protein, 9 aa, synthetic construct
GGQGNDHMD

SEQ ID NO: 37968 - protein, 9 aa, synthetic construct
GGQGNDHVI

SEQ ID NO: 37969 - protein, 9 aa, synthetic construct
GGQGNDHVS

SEQ ID NO: 37970 - protein, 9 aa, synthetic construct
GGQGNDIFQ

SEQ ID NO: 37971 - protein, 9 aa, synthetic construct
GGQGNDIFV

SEQ ID NO: 37972 - protein, 9 aa, synthetic construct
GGQGNDIIH

SEQ ID NO: 37973 - protein, 9 aa, synthetic construct
GGQGNDIII

SEQ ID NO: 37974 - protein, 9 aa, synthetic construct
GGQGNDDMT

SEQ ID NO: 37975 - protein, 9 aa, synthetic construct
GGQGNDDLW

SEQ ID NO: 37976 - protein, 9 aa, synthetic construct
GGQGLDTLY

SEQ ID NO: 37977 - protein, 9 aa, synthetic construct
GGQGNDALE

SEQ ID NO: 37978 - protein, 9 aa, synthetic construct
GGQGLDTMD

SEQ ID NO: 37979 - protein, 9 aa, synthetic construct
GGQGLDVIR

SEQ ID NO: 37980 - protein, 9 aa, synthetic construct
GGQGLDVLQ

SEQ ID NO: 37981 - protein, 9 aa, synthetic construct
GGQGLDWLR

SEQ ID NO: 37982 - protein, 9 aa, synthetic construct
GGQGLDYAD

SEQ ID NO: 37983 - protein, 9 aa, synthetic construct
GGQGLDYLE

SEQ ID NO: 37984 - protein, 9 aa, synthetic construct
GGQGMDFVD

SEQ ID NO: 37985 - protein, 9 aa, synthetic construct
GGQGMDLLF

SEQ ID NO: 37986 - protein, 9 aa, synthetic construct
GGQGMDMIF

SEQ ID NO: 37987 - protein, 9 aa, synthetic construct
GGQGMDQLL

SEQ ID NO: 37988 - protein, 9 aa, synthetic construct
GGQGMDQLS

SEQ ID NO: 37989 - protein, 9 aa, synthetic construct
GGQGMDYAD

SEQ ID NO: 37990 - protein, 9 aa, synthetic construct
GGQGNDAIV

SEQ ID NO: 37991 - protein, 9 aa, synthetic construct
GGQGNDALN

SEQ ID NO: 37992 - protein, 9 aa, synthetic construct
GGQGNDDLS

SEQ ID NO: 37993 - protein, 9 aa, synthetic construct
GGQGNDALR

SEQ ID NO: 37994 - protein, 9 aa, synthetic construct
GGQGNDALS

SEQ ID NO: 37995 - protein, 9 aa, synthetic construct
GGQGNDALV

SEQ ID NO: 37996 - protein, 9 aa, synthetic construct
GGQGNDAVF

SEQ ID NO: 37997 - protein, 9 aa, synthetic construct
GGQGNDAVT

SEQ ID NO: 37998 - protein, 9 aa, synthetic construct
GGQGNDAYL

SEQ ID NO: 37999 - protein, 9 aa, synthetic construct
GGQGNDDIN

SEQ ID NO: 38000 - protein, 9 aa, synthetic construct
GGQGNDDLE

SEQ ID NO: 38001 - protein, 9 aa, synthetic construct
GGQGNDDLK

SEQ ID NO: 38002 - protein, 9 aa, synthetic construct
GGQGNDDLL

SEQ ID NO: 38003 - protein, 9 aa, synthetic construct
GGQGNDDLN

SEQ ID NO: 38004 - protein, 9 aa, synthetic construct
GGQGNDDLQ

SEQ ID NO: 38005 - protein, 9 aa, synthetic construct
GGQGNDDLR

SEQ ID NO: 38006 - protein, 9 aa, synthetic construct
GGQGQDDLI

SEQ ID NO: 38007 - protein, 9 aa, synthetic construct
GGQGQDDVD

SEQ ID NO: 38008 - protein, 9 aa, synthetic construct
GGQGQDELG

SEQ ID NO: 38009 - protein, 9 aa, synthetic construct
GGQGSDQIF

SEQ ID NO: 38010 - protein, 9 aa, synthetic construct
GGQGSDVLY

SEQ ID NO: 38011 - protein, 9 aa, synthetic construct
GGQGSDVVL

SEQ ID NO: 38012 - protein, 9 aa, synthetic construct
GGQGSDVVV

SEQ ID NO: 38013 - protein, 9 aa, synthetic construct
GGQGSDVVY

SEQ ID NO: 38014 - protein, 9 aa, synthetic construct
GGQGSDVYI

SEQ ID NO: 38015 - protein, 9 aa, synthetic construct
GGQGSDWVF

SEQ ID NO: 38016 - protein, 9 aa, synthetic construct
GGQGSDYLF

SEQ ID NO: 38017 - protein, 9 aa, synthetic construct
GGQGSDYVD

SEQ ID NO: 38018 - protein, 9 aa, synthetic construct
GGQGTDALF

SEQ ID NO: 38019 - protein, 9 aa, synthetic construct
GGQGTDEIY

SEQ ID NO: 38020 - protein, 9 aa, synthetic construct
GGQGTDFAR

SEQ ID NO: 38021 - protein, 9 aa, synthetic construct
GGQGTDHLL

SEQ ID NO: 38022 - protein, 9 aa, synthetic construct
GGQGTDIAI

SEQ ID NO: 38023 - protein, 9 aa, synthetic construct
GGQGTDIAR

SEQ ID NO: 38024 - protein, 9 aa, synthetic construct
GGQGTDILD

SEQ ID NO: 38025 - protein, 9 aa, synthetic construct
GGQGTDIML

SEQ ID NO: 38026 - protein, 9 aa, synthetic construct
GGQGTDLLT

SEQ ID NO: 38027 - protein, 9 aa, synthetic construct
GGQGTDLVY

SEQ ID NO: 38028 - protein, 9 aa, synthetic construct
GGQGTDNLI

SEQ ID NO: 38029 - protein, 9 aa, synthetic construct
GGQGTDNVD

SEQ ID NO: 38030 - protein, 9 aa, synthetic construct
GGQGTDRFV

SEQ ID NO: 38031 - protein, 9 aa, synthetic construct
GGQGTDRLA

SEQ ID NO: 38032 - protein, 9 aa, synthetic construct
GGQGTDRLE

SEQ ID NO: 38033 - protein, 9 aa, synthetic construct
GGQGTDRLN

SEQ ID NO: 38034 - protein, 9 aa, synthetic construct
GGQGTDRLT

SEQ ID NO: 38035 - protein, 9 aa, synthetic construct
GGQGTDSIT

SEQ ID NO: 38036 - protein, 9 aa, synthetic construct
GGQGTDSLI

SEQ ID NO: 38037 - protein, 9 aa, synthetic construct
GGQGTDSLK

SEQ ID NO: 38038 - protein, 9 aa, synthetic construct
GGQGTDSLL

SEQ ID NO: 38039 - protein, 9 aa, synthetic construct
GGQGSDVLR

SEQ ID NO: 38040 - protein, 9 aa, synthetic construct
GGQGSDVLQ

SEQ ID NO: 38041 - protein, 9 aa, synthetic construct
GGQGSDVLN

SEQ ID NO: 38042 - protein, 9 aa, synthetic construct
GGQGSDTFN

SEQ ID NO: 38043 - protein, 9 aa, synthetic construct
GGQGSDQMR

SEQ ID NO: 38044 - protein, 9 aa, synthetic construct
GGQGSDRFW

SEQ ID NO: 38045 - protein, 9 aa, synthetic construct
GGQGSDRLD

SEQ ID NO: 38046 - protein, 9 aa, synthetic construct
GGQGSDRLL

SEQ ID NO: 38047 - protein, 9 aa, synthetic construct
GGQGSDRLY

SEQ ID NO: 38048 - protein, 9 aa, synthetic construct
GGQGSDRMW

SEQ ID NO: 38049 - protein, 9 aa, synthetic construct
GGQGSDSLI

SEQ ID NO: 38050 - protein, 9 aa, synthetic construct
GGQGSDSLV

SEQ ID NO: 38051 - protein, 9 aa, synthetic construct
GGQGSDSVN

SEQ ID NO: 38052 - protein, 9 aa, synthetic construct
GGQGSDSVY

SEQ ID NO: 38053 - protein, 9 aa, synthetic construct
GGQGSDTAS

SEQ ID NO: 38054 - protein, 9 aa, synthetic construct
GGQGSDTAV

SEQ ID NO: 38055 - protein, 9 aa, synthetic construct
GGQGSDTFD

SEQ ID NO: 38056 - protein, 9 aa, synthetic construct
GGQGSDTIT

SEQ ID NO: 38057 - protein, 9 aa, synthetic construct
GGQGSDVLA

SEQ ID NO: 38058 - protein, 9 aa, synthetic construct
GGQGSDTIY

SEQ ID NO: 38059 - protein, 9 aa, synthetic construct
GGQGSDTLS

SEQ ID NO: 38060 - protein, 9 aa, synthetic construct
GGQGSDTMA

SEQ ID NO: 38061 - protein, 9 aa, synthetic construct
GGQGSDTMT

SEQ ID NO: 38062 - protein, 9 aa, synthetic construct
GGQGSDTVL

SEQ ID NO: 38063 - protein, 9 aa, synthetic construct
GGQGSDTVM

SEQ ID NO: 38064 - protein, 9 aa, synthetic construct
GGQGSDTVY

SEQ ID NO: 38065 - protein, 9 aa, synthetic construct
GGQGSDTYR

SEQ ID NO: 38066 - protein, 9 aa, synthetic construct
GGQGSDTYY

SEQ ID NO: 38067 - protein, 9 aa, synthetic construct
GGQGSDVFR

SEQ ID NO: 38068 - protein, 9 aa, synthetic construct
GGQGSDVFV

SEQ ID NO: 38069 - protein, 9 aa, synthetic construct
GGQGSDVIE

SEQ ID NO: 38070 - protein, 9 aa, synthetic construct
GGQGSDVIY

SEQ ID NO: 38071 - protein, 9 aa, synthetic construct
GGQGTDSVF

SEQ ID NO: 38072 - protein, 9 aa, synthetic construct
GGQGTDSVQ

SEQ ID NO: 38073 - protein, 9 aa, synthetic construct
GGQGTDSVV

SEQ ID NO: 38074 - protein, 9 aa, synthetic construct
GGQGVDVLD

SEQ ID NO: 38075 - protein, 9 aa, synthetic construct
GGQGVDTIE

SEQ ID NO: 38076 - protein, 9 aa, synthetic construct
GGQGVDTIH

SEQ ID NO: 38077 - protein, 9 aa, synthetic construct
GGQGVDTIT

SEQ ID NO: 38078 - protein, 9 aa, synthetic construct
GGQGVDTIY

SEQ ID NO: 38079 - protein, 9 aa, synthetic construct
GGQGVDTLA

SEQ ID NO: 38080 - protein, 9 aa, synthetic construct
GGQGVDTLK

SEQ ID NO: 38081 - protein, 9 aa, synthetic construct
GGQGVDTLL

SEQ ID NO: 38082 - protein, 9 aa, synthetic construct
GGQGVDTLN

SEQ ID NO: 38083 - protein, 9 aa, synthetic construct
GGQGVDTLR

SEQ ID NO: 38084 - protein, 9 aa, synthetic construct
GGQGVDTLS

SEQ ID NO: 38085 - protein, 9 aa, synthetic construct
GGQGVDTMS

SEQ ID NO: 38086 - protein, 9 aa, synthetic construct
GGQGVDTMY

SEQ ID NO: 38087 - protein, 9 aa, synthetic construct
GGQGVDTVF

SEQ ID NO: 38088 - protein, 9 aa, synthetic construct
GGQGVDVLE

SEQ ID NO: 38089 - protein, 9 aa, synthetic construct
GGQGVDSMS

SEQ ID NO: 38090 - protein, 9 aa, synthetic construct
GGQGVDVMT

SEQ ID NO: 38091 - protein, 9 aa, synthetic construct
GGQGVDVVR

SEQ ID NO: 38092 - protein, 9 aa, synthetic construct
GGQGVDWVY

SEQ ID NO: 38093 - protein, 9 aa, synthetic construct
GGQGVDYID

SEQ ID NO: 38094 - protein, 9 aa, synthetic construct
GGQGWDNIR

SEQ ID NO: 38095 - protein, 9 aa, synthetic construct
GGQGWDTLY

SEQ ID NO: 38096 - protein, 9 aa, synthetic construct
GGQGWDVIG

SEQ ID NO: 38097 - protein, 9 aa, synthetic construct
GGQGWDYLS

SEQ ID NO: 38098 - protein, 9 aa, synthetic construct
GGQGXDTIL

SEQ ID NO: 38099 - protein, 9 aa, synthetic construct
GGQGYDLLE

SEQ ID NO: 38100 - protein, 9 aa, synthetic construct
GGQGYDNLY

SEQ ID NO: 38101 - protein, 9 aa, synthetic construct
GGQGYDRLT

SEQ ID NO: 38102 - protein, 9 aa, synthetic construct
GGQGYDRLY

SEQ ID NO: 38103 - protein, 9 aa, synthetic construct
GGQGVDTID

SEQ ID NO: 38104 - protein, 9 aa, synthetic construct
GGQGVDSMI

SEQ ID NO: 38105 - protein, 9 aa, synthetic construct
GGQGTDTAD

SEQ ID NO: 38106 - protein, 9 aa, synthetic construct
GGQGTDWLA

SEQ ID NO: 38107 - protein, 9 aa, synthetic construct
GGQGTDTIQ

SEQ ID NO: 38108 - protein, 9 aa, synthetic construct
GGQGTDTIT

SEQ ID NO: 38109 - protein, 9 aa, synthetic construct
GGQGTDTIW

SEQ ID NO: 38110 - protein, 9 aa, synthetic construct
GGQGTDTLF

SEQ ID NO: 38111 - protein, 9 aa, synthetic construct
GGQGTDTLI

SEQ ID NO: 38112 - protein, 9 aa, synthetic construct
GGQGTDTLN

SEQ ID NO: 38113 - protein, 9 aa, synthetic construct
GGQGTDTLQ

SEQ ID NO: 38114 - protein, 9 aa, synthetic construct
GGQGTDTVF

SEQ ID NO: 38115 - protein, 9 aa, synthetic construct
GGQGTDTVR

SEQ ID NO: 38116 - protein, 9 aa, synthetic construct
GGQGTDVLD

SEQ ID NO: 38117 - protein, 9 aa, synthetic construct
GGQGTDVLE

SEQ ID NO: 38118 - protein, 9 aa, synthetic construct
GGQGTDVLI

SEQ ID NO: 38119 - protein, 9 aa, synthetic construct
GGQGTDVLS

SEQ ID NO: 38120 - protein, 9 aa, synthetic construct
GGQGVDALF

SEQ ID NO: 38121 - protein, 9 aa, synthetic construct
GGQGVDSLN

SEQ ID NO: 38122 - protein, 9 aa, synthetic construct
GGQGVDELD

SEQ ID NO: 38123 - protein, 9 aa, synthetic construct
GGQGVDKLF

SEQ ID NO: 38124 - protein, 9 aa, synthetic construct
GGQGVDLLK

SEQ ID NO: 38125 - protein, 9 aa, synthetic construct
GGQGVDLLV

SEQ ID NO: 38126 - protein, 9 aa, synthetic construct
GGQGVDLVY

SEQ ID NO: 38127 - protein, 9 aa, synthetic construct
GGQGVDMLT

SEQ ID NO: 38128 - protein, 9 aa, synthetic construct
GGQGVDRAT

SEQ ID NO: 38129 - protein, 9 aa, synthetic construct
GGQGVDRIG

SEQ ID NO: 38130 - protein, 9 aa, synthetic construct
GGQGVDRLD

SEQ ID NO: 38131 - protein, 9 aa, synthetic construct
GGQGVDRLE

SEQ ID NO: 38132 - protein, 9 aa, synthetic construct
GGQGVDSIA

SEQ ID NO: 38133 - protein, 9 aa, synthetic construct
GGQGVDSLI

SEQ ID NO: 38134 - protein, 9 aa, synthetic construct
GGQGVDSLL

SEQ ID NO: 38135 - protein, 9 aa, synthetic construct
GGQGSDQLY

SEQ ID NO: 38136 - protein, 9 aa, synthetic construct
GGQGSDMLT

SEQ ID NO: 38137 - protein, 9 aa, synthetic construct
GGQGQDELK

SEQ ID NO: 38138 - protein, 9 aa, synthetic construct
GGQGSDMAV

SEQ ID NO: 38139 - protein, 9 aa, synthetic construct
GGQGQDYAD

SEQ ID NO: 38140 - protein, 9 aa, synthetic construct
GGQGQDYLD

SEQ ID NO: 38141 - protein, 9 aa, synthetic construct
GGQGQDYLS

SEQ ID NO: 38142 - protein, 9 aa, synthetic construct
GGQGRDALN

SEQ ID NO: 38143 - protein, 9 aa, synthetic construct
GGQGRDALY

SEQ ID NO: 38144 - protein, 9 aa, synthetic construct
GGQGRDDLA

SEQ ID NO: 38145 - protein, 9 aa, synthetic construct
GGQGRDDLS

SEQ ID NO: 38146 - protein, 9 aa, synthetic construct
GGQGRDELF

SEQ ID NO: 38147 - protein, 9 aa, synthetic construct
GGQGRDELW

SEQ ID NO: 38148 - protein, 9 aa, synthetic construct
GGQGRDEMH

SEQ ID NO: 38149 - protein, 9 aa, synthetic construct
GGQGRDEVI

SEQ ID NO: 38150 - protein, 9 aa, synthetic construct
GGQGRDHLA

SEQ ID NO: 38151 - protein, 9 aa, synthetic construct
GGQGRDHLR

SEQ ID NO: 38152 - protein, 9 aa, synthetic construct
GGQGRDHMF

SEQ ID NO: 38153 - protein, 9 aa, synthetic construct
GGQGRDILI

SEQ ID NO: 38154 - protein, 9 aa, synthetic construct
GGQGRDILR

SEQ ID NO: 38155 - protein, 9 aa, synthetic construct
GGQGRDIMS

SEQ ID NO: 38156 - protein, 9 aa, synthetic construct
GGQGRDIVR

SEQ ID NO: 38157 - protein, 9 aa, synthetic construct
GGQGRDKLD

SEQ ID NO: 38158 - protein, 9 aa, synthetic construct
GGQGRDKLS

SEQ ID NO: 38159 - protein, 9 aa, synthetic construct
GGQGRDLAA

SEQ ID NO: 38160 - protein, 9 aa, synthetic construct
GGQGRDLFV

SEQ ID NO: 38161 - protein, 9 aa, synthetic construct
GGQGRDLLI

SEQ ID NO: 38162 - protein, 9 aa, synthetic construct
GGQGRDLLL

SEQ ID NO: 38163 - protein, 9 aa, synthetic construct
GGQGRDLLV

SEQ ID NO: 38164 - protein, 9 aa, synthetic construct
GGQGRDLLY

SEQ ID NO: 38165 - protein, 9 aa, synthetic construct
GGQGRDMLF

SEQ ID NO: 38166 - protein, 9 aa, synthetic construct
GGQGRDQIF

SEQ ID NO: 38167 - protein, 9 aa, synthetic construct
GGQGRDQLG

SEQ ID NO: 38168 - protein, 9 aa, synthetic construct
GGQGQDVMS

SEQ ID NO: 38169 - protein, 9 aa, synthetic construct
GGQGQDVLT

SEQ ID NO: 38170 - protein, 9 aa, synthetic construct
GGQGQDVLI

SEQ ID NO: 38171 - protein, 9 aa, synthetic construct
GGQGQDSFV

SEQ ID NO: 38172 - protein, 9 aa, synthetic construct
GGQGQDHIV

SEQ ID NO: 38173 - protein, 9 aa, synthetic construct
GGQGQDIFV

SEQ ID NO: 38174 - protein, 9 aa, synthetic construct
GGQGQDILH

SEQ ID NO: 38175 - protein, 9 aa, synthetic construct
GGQGQDILT

SEQ ID NO: 38176 - protein, 9 aa, synthetic construct
GGQGQDLFI

SEQ ID NO: 38177 - protein, 9 aa, synthetic construct
GGQGQDLIR

SEQ ID NO: 38178 - protein, 9 aa, synthetic construct
GGQGQDLVY

SEQ ID NO: 38179 - protein, 9 aa, synthetic construct
GGQGQDMIR

SEQ ID NO: 38180 - protein, 9 aa, synthetic construct
GGQGQDMLM

SEQ ID NO: 38181 - protein, 9 aa, synthetic construct
GGQGQDQLT

SEQ ID NO: 38182 - protein, 9 aa, synthetic construct
GGQGQDQLY

SEQ ID NO: 38183 - protein, 9 aa, synthetic construct
GGQGQDRID

SEQ ID NO: 38184 - protein, 9 aa, synthetic construct
GGQGQDRLV

SEQ ID NO: 38185 - protein, 9 aa, synthetic construct
GGQGQDSIA

SEQ ID NO: 38186 - protein, 9 aa, synthetic construct
GGQGQDVLD

SEQ ID NO: 38187 - protein, 9 aa, synthetic construct
GGQGQDSLF

SEQ ID NO: 38188 - protein, 9 aa, synthetic construct
GGQGQDSLN

SEQ ID NO: 38189 - protein, 9 aa, synthetic construct
GGQGQDSLV

SEQ ID NO: 38190 - protein, 9 aa, synthetic construct
GGQGQDSLY

SEQ ID NO: 38191 - protein, 9 aa, synthetic construct
GGQGQDTFK

SEQ ID NO: 38192 - protein, 9 aa, synthetic construct
GGQGQDTID

SEQ ID NO: 38193 - protein, 9 aa, synthetic construct
GGQGQDTIS

SEQ ID NO: 38194 - protein, 9 aa, synthetic construct
GGQGQDTIY

SEQ ID NO: 38195 - protein, 9 aa, synthetic construct
GGQGQDTLG

SEQ ID NO: 38196 - protein, 9 aa, synthetic construct
GGQGQDTLL

SEQ ID NO: 38197 - protein, 9 aa, synthetic construct
GGQGQDTLT

SEQ ID NO: 38198 - protein, 9 aa, synthetic construct
GGQGQDTMT

SEQ ID NO: 38199 - protein, 9 aa, synthetic construct
GGQGQDVFV

SEQ ID NO: 38200 - protein, 9 aa, synthetic construct
GGQGRDQLS

SEQ ID NO: 38201 - protein, 9 aa, synthetic construct
GGQGRDRIL

SEQ ID NO: 38202 - protein, 9 aa, synthetic construct
GGQGRDRLD

SEQ ID NO: 38203 - protein, 9 aa, synthetic construct
GGQGSDHLS

SEQ ID NO: 38204 - protein, 9 aa, synthetic construct
GGQGSDDLR

SEQ ID NO: 38205 - protein, 9 aa, synthetic construct
GGQGSDDLS

SEQ ID NO: 38206 - protein, 9 aa, synthetic construct
GGQGSDDMY

SEQ ID NO: 38207 - protein, 9 aa, synthetic construct
GGQGSDELL

SEQ ID NO: 38208 - protein, 9 aa, synthetic construct
GGQGSDELY

SEQ ID NO: 38209 - protein, 9 aa, synthetic construct
GGQGSDEVS

SEQ ID NO: 38210 - protein, 9 aa, synthetic construct
GGQGSDFIY

SEQ ID NO: 38211 - protein, 9 aa, synthetic construct
GGQGSDFLD

SEQ ID NO: 38212 - protein, 9 aa, synthetic construct
GGQGSDFLH

SEQ ID NO: 38213 - protein, 9 aa, synthetic construct
GGQGSDFVY

SEQ ID NO: 38214 - protein, 9 aa, synthetic construct
GGQGSDHIY

SEQ ID NO: 38215 - protein, 9 aa, synthetic construct
GGQGSDHLD

SEQ ID NO: 38216 - protein, 9 aa, synthetic construct
GGQGSDHLE

SEQ ID NO: 38217 - protein, 9 aa, synthetic construct
GGQGSDIFG

SEQ ID NO: 38218 - protein, 9 aa, synthetic construct
GGQGSDAVY

SEQ ID NO: 38219 - protein, 9 aa, synthetic construct
GGQGSDILD

SEQ ID NO: 38220 - protein, 9 aa, synthetic construct
GGQGSDILY

SEQ ID NO: 38221 - protein, 9 aa, synthetic construct
GGQGSDIVV

SEQ ID NO: 38222 - protein, 9 aa, synthetic construct
GGQGSDIYD

SEQ ID NO: 38223 - protein, 9 aa, synthetic construct
GGQGSDKVF

SEQ ID NO: 38224 - protein, 9 aa, synthetic construct
GGQGSDLFL

SEQ ID NO: 38225 - protein, 9 aa, synthetic construct
GGQGSDLIF

SEQ ID NO: 38226 - protein, 9 aa, synthetic construct
GGQGSDLIY

SEQ ID NO: 38227 - protein, 9 aa, synthetic construct
GGQGSDLLK

SEQ ID NO: 38228 - protein, 9 aa, synthetic construct
GGQGSDLLN

SEQ ID NO: 38229 - protein, 9 aa, synthetic construct
GGQGSDLVL

SEQ ID NO: 38230 - protein, 9 aa, synthetic construct
GGQGSDLVY

SEQ ID NO: 38231 - protein, 9 aa, synthetic construct
GGQGSDLYV

SEQ ID NO: 38232 - protein, 9 aa, synthetic construct
GGQGSDDLL

SEQ ID NO: 38233 - protein, 9 aa, synthetic construct
GGQGSDALF

SEQ ID NO: 38234 - protein, 9 aa, synthetic construct
GGQGRDRLL

SEQ ID NO: 38235 - protein, 9 aa, synthetic construct
GGQGRDTLL

SEQ ID NO: 38236 - protein, 9 aa, synthetic construct
GGQGRDRLM

SEQ ID NO: 38237 - protein, 9 aa, synthetic construct
GGQGRDRLT

SEQ ID NO: 38238 - protein, 9 aa, synthetic construct
GGQGRDRLY

SEQ ID NO: 38239 - protein, 9 aa, synthetic construct
GGQGRDSIE

SEQ ID NO: 38240 - protein, 9 aa, synthetic construct
GGQGRDSLE

SEQ ID NO: 38241 - protein, 9 aa, synthetic construct
GGQGRDSLI

SEQ ID NO: 38242 - protein, 9 aa, synthetic construct
GGQGRDSLK

SEQ ID NO: 38243 - protein, 9 aa, synthetic construct
GGQGRDSLT

SEQ ID NO: 38244 - protein, 9 aa, synthetic construct
GGQGRDSLV

SEQ ID NO: 38245 - protein, 9 aa, synthetic construct
GGQGRDTFT

SEQ ID NO: 38246 - protein, 9 aa, synthetic construct
GGQGRDTIE

SEQ ID NO: 38247 - protein, 9 aa, synthetic construct
GGQGRDTIF

SEQ ID NO: 38248 - protein, 9 aa, synthetic construct
GGQGRDTIN

SEQ ID NO: 38249 - protein, 9 aa, synthetic construct
GGQGRDTLR

SEQ ID NO: 38250 - protein, 9 aa, synthetic construct
GGQGSDAIH

SEQ ID NO: 38251 - protein, 9 aa, synthetic construct
GGQGRDTLT

SEQ ID NO: 38252 - protein, 9 aa, synthetic construct
GGQGRDTLY

SEQ ID NO: 38253 - protein, 9 aa, synthetic construct
GGQGRDTMW

SEQ ID NO: 38254 - protein, 9 aa, synthetic construct
GGQGRDTYI

SEQ ID NO: 38255 - protein, 9 aa, synthetic construct
GGQGRDVFS

SEQ ID NO: 38256 - protein, 9 aa, synthetic construct
GGQGRDVFV

SEQ ID NO: 38257 - protein, 9 aa, synthetic construct
GGQGRDVIE

SEQ ID NO: 38258 - protein, 9 aa, synthetic construct
GGQGRDVLI

SEQ ID NO: 38259 - protein, 9 aa, synthetic construct
GGQGRDVLN

SEQ ID NO: 38260 - protein, 9 aa, synthetic construct
GGQGRDVMV

SEQ ID NO: 38261 - protein, 9 aa, synthetic construct
GGQGRDYIE

SEQ ID NO: 38262 - protein, 9 aa, synthetic construct
GGQGRDYIT

SEQ ID NO: 38263 - protein, 9 aa, synthetic construct
GGQGSDAAS

SEQ ID NO: 38264 - protein, 9 aa, synthetic construct
GGSGRDLLF

SEQ ID NO: 38265 - protein, 9 aa, synthetic construct
GGSGRDLLL

SEQ ID NO: 38266 - protein, 9 aa, synthetic construct
GGPGDDTII

SEQ ID NO: 38267 - protein, 9 aa, synthetic construct
GGVGHDLVT

SEQ ID NO: 38268 - protein, 9 aa, synthetic construct
GGVGGDLLL

SEQ ID NO: 38269 - protein, 9 aa, synthetic construct
GGVGGDLLR

SEQ ID NO: 38270 - protein, 9 aa, synthetic construct
GGVGGDRLE

SEQ ID NO: 38271 - protein, 9 aa, synthetic construct
GGVGGDRMQ

SEQ ID NO: 38272 - protein, 9 aa, synthetic construct
GGVGGDSIA

SEQ ID NO: 38273 - protein, 9 aa, synthetic construct
GGVGGDSIT

SEQ ID NO: 38274 - protein, 9 aa, synthetic construct
GGVGGDSLI

SEQ ID NO: 38275 - protein, 9 aa, synthetic construct
GGVGGDSLN

SEQ ID NO: 38276 - protein, 9 aa, synthetic construct
GGVGGDTFE

SEQ ID NO: 38277 - protein, 9 aa, synthetic construct
GGVGGDTFT

SEQ ID NO: 38278 - protein, 9 aa, synthetic construct
GGVGGDTFV

SEQ ID NO: 38279 - protein, 9 aa, synthetic construct
GGVGGDTIY

SEQ ID NO: 38280 - protein, 9 aa, synthetic construct
GGVGGDTLD

SEQ ID NO: 38281 - protein, 9 aa, synthetic construct
GGVGGDTMS

SEQ ID NO: 38282 - protein, 9 aa, synthetic construct
GGVGGDVIS

SEQ ID NO: 38283 - protein, 9 aa, synthetic construct
GGVGGDVLI

SEQ ID NO: 38284 - protein, 9 aa, synthetic construct
GGVGGDVLR

SEQ ID NO: 38285 - protein, 9 aa, synthetic construct
GGVGGDYLA

SEQ ID NO: 38286 - protein, 9 aa, synthetic construct
GGVGHDALI

SEQ ID NO: 38287 - protein, 9 aa, synthetic construct
GGVGHDDIY

SEQ ID NO: 38288 - protein, 9 aa, synthetic construct
GGVGHDHLS

SEQ ID NO: 38289 - protein, 9 aa, synthetic construct
GGVGHDILD

SEQ ID NO: 38290 - protein, 9 aa, synthetic construct
GGVGHDILG

SEQ ID NO: 38291 - protein, 9 aa, synthetic construct
GGVGHDILI

SEQ ID NO: 38292 - protein, 9 aa, synthetic construct
GGVGHDILN

SEQ ID NO: 38293 - protein, 9 aa, synthetic construct
GGVGHDIVV

SEQ ID NO: 38294 - protein, 9 aa, synthetic construct
GGVGHDKLM

SEQ ID NO: 38295 - protein, 9 aa, synthetic construct
GGVGHDKLY

SEQ ID NO: 38296 - protein, 9 aa, synthetic construct
GGVGHDLIE

SEQ ID NO: 38297 - protein, 9 aa, synthetic construct
GGVGGDLLG

SEQ ID NO: 38298 - protein, 9 aa, synthetic construct
GGVGGDHLI

SEQ ID NO: 38299 - protein, 9 aa, synthetic construct
GGVGGDHLD

SEQ ID NO: 38300 - protein, 9 aa, synthetic construct
GGVGFDLID

SEQ ID NO: 38301 - protein, 9 aa, synthetic construct
GGVGEDRLY

SEQ ID NO: 38302 - protein, 9 aa, synthetic construct
GGVGEDSFV

SEQ ID NO: 38303 - protein, 9 aa, synthetic construct
GGVGEDTIM

SEQ ID NO: 38304 - protein, 9 aa, synthetic construct
GGVGEDTLK

SEQ ID NO: 38305 - protein, 9 aa, synthetic construct
GGVGEDTLN

SEQ ID NO: 38306 - protein, 9 aa, synthetic construct
GGVGEDTMT

SEQ ID NO: 38307 - protein, 9 aa, synthetic construct
GGVGEDVIS

SEQ ID NO: 38308 - protein, 9 aa, synthetic construct
GGVGEDVLD

SEQ ID NO: 38309 - protein, 9 aa, synthetic construct
GGVGFDAIS

SEQ ID NO: 38310 - protein, 9 aa, synthetic construct
GGVGFDALS

SEQ ID NO: 38311 - protein, 9 aa, synthetic construct
GGVGFDIAD

SEQ ID NO: 38312 - protein, 9 aa, synthetic construct
GGVGFDIFV

SEQ ID NO: 38313 - protein, 9 aa, synthetic construct
GGVGFDLAD

SEQ ID NO: 38314 - protein, 9 aa, synthetic construct
GGVGFDLLR

SEQ ID NO: 38315 - protein, 9 aa, synthetic construct
GGVGGDFLQ

SEQ ID NO: 38316 - protein, 9 aa, synthetic construct
GGVGFDLVT

SEQ ID NO: 38317 - protein, 9 aa, synthetic construct
GGVGFDQVS

SEQ ID NO: 38318 - protein, 9 aa, synthetic construct
GGVGFDRAD

SEQ ID NO: 38319 - protein, 9 aa, synthetic construct
GGVGFDTFV

SEQ ID NO: 38320 - protein, 9 aa, synthetic construct
GGVGFDTLD

SEQ ID NO: 38321 - protein, 9 aa, synthetic construct
GGVGFDTLL

SEQ ID NO: 38322 - protein, 9 aa, synthetic construct
GGVGFDVLD

SEQ ID NO: 38323 - protein, 9 aa, synthetic construct
GGVGFDVLE

SEQ ID NO: 38324 - protein, 9 aa, synthetic construct
GGVGFDVLR

SEQ ID NO: 38325 - protein, 9 aa, synthetic construct
GGVGFDVLT

SEQ ID NO: 38326 - protein, 9 aa, synthetic construct
GGVGFDVMI

SEQ ID NO: 38327 - protein, 9 aa, synthetic construct
GGVGFDWMT

SEQ ID NO: 38328 - protein, 9 aa, synthetic construct
GGVGGDFLD

SEQ ID NO: 38329 - protein, 9 aa, synthetic construct
GGVGHDLLS

SEQ ID NO: 38330 - protein, 9 aa, synthetic construct
GGVGHDMLD

SEQ ID NO: 38331 - protein, 9 aa, synthetic construct
GGVGKDRLV

SEQ ID NO: 38332 - protein, 9 aa, synthetic construct
GGVGHDMLV

SEQ ID NO: 38333 - protein, 9 aa, synthetic construct
GGVGIDKLT

SEQ ID NO: 38334 - protein, 9 aa, synthetic construct
GGVGIDKMT

SEQ ID NO: 38335 - protein, 9 aa, synthetic construct
GGVGIDNIS

SEQ ID NO: 38336 - protein, 9 aa, synthetic construct
GGVGIDNLG

SEQ ID NO: 38337 - protein, 9 aa, synthetic construct
GGVGIDQFF

SEQ ID NO: 38338 - protein, 9 aa, synthetic construct
GGVGIDQLW

SEQ ID NO: 38339 - protein, 9 aa, synthetic construct
GGVGIDQMA

SEQ ID NO: 38340 - protein, 9 aa, synthetic construct
GGVGIDRLY

SEQ ID NO: 38341 - protein, 9 aa, synthetic construct
GGVGIDSAN

SEQ ID NO: 38342 - protein, 9 aa, synthetic construct
GGVGIDSLL

SEQ ID NO: 38343 - protein, 9 aa, synthetic construct
GGVGIDSLY

SEQ ID NO: 38344 - protein, 9 aa, synthetic construct
GGVGIDTAH

SEQ ID NO: 38345 - protein, 9 aa, synthetic construct
GGVGIDTLA

SEQ ID NO: 38346 - protein, 9 aa, synthetic construct
GGVGIDTLD

SEQ ID NO: 38347 - protein, 9 aa, synthetic construct
GGVGIDTVS

SEQ ID NO: 38348 - protein, 9 aa, synthetic construct
GGVGIDVLN

SEQ ID NO: 38349 - protein, 9 aa, synthetic construct
GGVGIDWVS

SEQ ID NO: 38350 - protein, 9 aa, synthetic construct
GGVGKDAFR

SEQ ID NO: 38351 - protein, 9 aa, synthetic construct
GGVGKDALD

SEQ ID NO: 38352 - protein, 9 aa, synthetic construct
GGVGKDGLF

SEQ ID NO: 38353 - protein, 9 aa, synthetic construct
GGVGKDIMS

SEQ ID NO: 38354 - protein, 9 aa, synthetic construct
GGVGKDKID

SEQ ID NO: 38355 - protein, 9 aa, synthetic construct
GGVGKDKLL

SEQ ID NO: 38356 - protein, 9 aa, synthetic construct
GGVGKDKLN

SEQ ID NO: 38357 - protein, 9 aa, synthetic construct
GGVGKDLFK

SEQ ID NO: 38358 - protein, 9 aa, synthetic construct
GGVGKDNLF

SEQ ID NO: 38359 - protein, 9 aa, synthetic construct
GGVGKDNLG

SEQ ID NO: 38360 - protein, 9 aa, synthetic construct
GGVGKDRID

SEQ ID NO: 38361 - protein, 9 aa, synthetic construct
GGVGKDRLD

SEQ ID NO: 38362 - protein, 9 aa, synthetic construct
GGVGIDKIS

SEQ ID NO: 38363 - protein, 9 aa, synthetic construct
GGVGIDKIF

SEQ ID NO: 38364 - protein, 9 aa, synthetic construct
GGVGIDKAF

SEQ ID NO: 38365 - protein, 9 aa, synthetic construct
GGVGHDTYV

SEQ ID NO: 38366 - protein, 9 aa, synthetic construct
GGVGHDNID

SEQ ID NO: 38367 - protein, 9 aa, synthetic construct
GGVGHDQLL

SEQ ID NO: 38368 - protein, 9 aa, synthetic construct
GGVGHDRLL

SEQ ID NO: 38369 - protein, 9 aa, synthetic construct
GGVGHDRLV

SEQ ID NO: 38370 - protein, 9 aa, synthetic construct
GGVGHDRLY

SEQ ID NO: 38371 - protein, 9 aa, synthetic construct
GGVGHDSIL

SEQ ID NO: 38372 - protein, 9 aa, synthetic construct
GGVGHDSLI

SEQ ID NO: 38373 - protein, 9 aa, synthetic construct
GGVGHDSLY

SEQ ID NO: 38374 - protein, 9 aa, synthetic construct
GGVGHDSVS

SEQ ID NO: 38375 - protein, 9 aa, synthetic construct
GGVGHDTLL

SEQ ID NO: 38376 - protein, 9 aa, synthetic construct
GGVGHDTLM

SEQ ID NO: 38377 - protein, 9 aa, synthetic construct
GGVGHDTLT

SEQ ID NO: 38378 - protein, 9 aa, synthetic construct
GGVGHDTYE

SEQ ID NO: 38379 - protein, 9 aa, synthetic construct
GGVGHDVFV

SEQ ID NO: 38380 - protein, 9 aa, synthetic construct
GGVGIDILK

SEQ ID NO: 38381 - protein, 9 aa, synthetic construct
GGVGHDVIS

SEQ ID NO: 38382 - protein, 9 aa, synthetic construct
GGVGHDVIV

SEQ ID NO: 38383 - protein, 9 aa, synthetic construct
GGVGHDVLE

SEQ ID NO: 38384 - protein, 9 aa, synthetic construct
GGVGHDVLQ

SEQ ID NO: 38385 - protein, 9 aa, synthetic construct
GGVGHDVVK

SEQ ID NO: 38386 - protein, 9 aa, synthetic construct
GGVGHDYAS

SEQ ID NO: 38387 - protein, 9 aa, synthetic construct
GGVGIDALA

SEQ ID NO: 38388 - protein, 9 aa, synthetic construct
GGVGIDALF

SEQ ID NO: 38389 - protein, 9 aa, synthetic construct
GGVGIDAML

SEQ ID NO: 38390 - protein, 9 aa, synthetic construct
GGVGIDFLI

SEQ ID NO: 38391 - protein, 9 aa, synthetic construct
GGVGIDGLT

SEQ ID NO: 38392 - protein, 9 aa, synthetic construct
GGVGIDIID

SEQ ID NO: 38393 - protein, 9 aa, synthetic construct
GGVGIDILF

SEQ ID NO: 38394 - protein, 9 aa, synthetic construct
GGVGEDRLE

SEQ ID NO: 38395 - protein, 9 aa, synthetic construct
GGVGEDQLH

SEQ ID NO: 38396 - protein, 9 aa, synthetic construct
GGVGEDNLY

SEQ ID NO: 38397 - protein, 9 aa, synthetic construct
GGVGEDLLR

SEQ ID NO: 38398 - protein, 9 aa, synthetic construct
GGVGDDNYH

SEQ ID NO: 38399 - protein, 9 aa, synthetic construct
GGVGDDQIW

SEQ ID NO: 38400 - protein, 9 aa, synthetic construct
GGVGDDQLA

SEQ ID NO: 38401 - protein, 9 aa, synthetic construct
GGVGDDQML

SEQ ID NO: 38402 - protein, 9 aa, synthetic construct
GGVGDDQVF

SEQ ID NO: 38403 - protein, 9 aa, synthetic construct
GGVGDDQVS

SEQ ID NO: 38404 - protein, 9 aa, synthetic construct
GGVGDDQVY

SEQ ID NO: 38405 - protein, 9 aa, synthetic construct
GGVGDDQYF

SEQ ID NO: 38406 - protein, 9 aa, synthetic construct
GGVGDDRAE

SEQ ID NO: 38407 - protein, 9 aa, synthetic construct
GGVGDDRIE

SEQ ID NO: 38408 - protein, 9 aa, synthetic construct
GGVGDDRLD

SEQ ID NO: 38409 - protein, 9 aa, synthetic construct
GGVGDDRLG

SEQ ID NO: 38410 - protein, 9 aa, synthetic construct
GGVGDDRLQ

SEQ ID NO: 38411 - protein, 9 aa, synthetic construct
GGVGDDRLR

SEQ ID NO: 38412 - protein, 9 aa, synthetic construct
GGVGDDRLT

SEQ ID NO: 38413 - protein, 9 aa, synthetic construct
GGVGDDRLW

SEQ ID NO: 38414 - protein, 9 aa, synthetic construct
GGVGDDRMG

SEQ ID NO: 38415 - protein, 9 aa, synthetic construct
GGVGDDRMW

SEQ ID NO: 38416 - protein, 9 aa, synthetic construct
GGVGDDRMY

SEQ ID NO: 38417 - protein, 9 aa, synthetic construct
GGVGDDRVE

SEQ ID NO: 38418 - protein, 9 aa, synthetic construct
GGVGDDRVI

SEQ ID NO: 38419 - protein, 9 aa, synthetic construct
GGVGDDRYL

SEQ ID NO: 38420 - protein, 9 aa, synthetic construct
GGVGDDRYR

SEQ ID NO: 38421 - protein, 9 aa, synthetic construct
GGVGDDRYY

SEQ ID NO: 38422 - protein, 9 aa, synthetic construct
GGVGDDSAD

SEQ ID NO: 38423 - protein, 9 aa, synthetic construct
GGVGDDSFL

SEQ ID NO: 38424 - protein, 9 aa, synthetic construct
GGVGDDSIF

SEQ ID NO: 38425 - protein, 9 aa, synthetic construct
GGVGDDSIG

SEQ ID NO: 38426 - protein, 9 aa, synthetic construct
GGVGDDSIQ

SEQ ID NO: 38427 - protein, 9 aa, synthetic construct
GGVGDDNVA

SEQ ID NO: 38428 - protein, 9 aa, synthetic construct
GGVGDDNMN

SEQ ID NO: 38429 - protein, 9 aa, synthetic construct
GGVGDDNLN

SEQ ID NO: 38430 - protein, 9 aa, synthetic construct
GGVGDDLLT

SEQ ID NO: 38431 - protein, 9 aa, synthetic construct
GGVGDDKVE

SEQ ID NO: 38432 - protein, 9 aa, synthetic construct
GGVGDDKVS

SEQ ID NO: 38433 - protein, 9 aa, synthetic construct
GGVGDDLAI

SEQ ID NO: 38434 - protein, 9 aa, synthetic construct
GGVGDDLFM

SEQ ID NO: 38435 - protein, 9 aa, synthetic construct
GGVGDDLFV

SEQ ID NO: 38436 - protein, 9 aa, synthetic construct
GGVGDDLFY

SEQ ID NO: 38437 - protein, 9 aa, synthetic construct
GGVGDDLIT

SEQ ID NO: 38438 - protein, 9 aa, synthetic construct
GGVGDDLIY

SEQ ID NO: 38439 - protein, 9 aa, synthetic construct
GGVGDDLLE

SEQ ID NO: 38440 - protein, 9 aa, synthetic construct
GGVGDDLLH

SEQ ID NO: 38441 - protein, 9 aa, synthetic construct
GGVGDDLLK

SEQ ID NO: 38442 - protein, 9 aa, synthetic construct
GGVGDDLLL

SEQ ID NO: 38443 - protein, 9 aa, synthetic construct
GGVGDDLLR

SEQ ID NO: 38444 - protein, 9 aa, synthetic construct
GGVGDDLLW

SEQ ID NO: 38445 - protein, 9 aa, synthetic construct
GGVGDDNLD

SEQ ID NO: 38446 - protein, 9 aa, synthetic construct
GGVGDDLME

SEQ ID NO: 38447 - protein, 9 aa, synthetic construct
GGVGDDLMI

SEQ ID NO: 38448 - protein, 9 aa, synthetic construct
GGVGDDLMS

SEQ ID NO: 38449 - protein, 9 aa, synthetic construct
GGVGDDLMT

SEQ ID NO: 38450 - protein, 9 aa, synthetic construct
GGVGDDLVT

SEQ ID NO: 38451 - protein, 9 aa, synthetic construct
GGVGDDLYL

SEQ ID NO: 38452 - protein, 9 aa, synthetic construct
GGVGDDLYR

SEQ ID NO: 38453 - protein, 9 aa, synthetic construct
GGVGDDMFL

SEQ ID NO: 38454 - protein, 9 aa, synthetic construct
GGVGDDNFT

SEQ ID NO: 38455 - protein, 9 aa, synthetic construct
GGVGDDNID

SEQ ID NO: 38456 - protein, 9 aa, synthetic construct
GGVGDDNIG

SEQ ID NO: 38457 - protein, 9 aa, synthetic construct
GGVGDDNIN

SEQ ID NO: 38458 - protein, 9 aa, synthetic construct
GGVGDDNIY

SEQ ID NO: 38459 - protein, 9 aa, synthetic construct
GGVGDDSIR

SEQ ID NO: 38460 - protein, 9 aa, synthetic construct
GGVGDDSLF

SEQ ID NO: 38461 - protein, 9 aa, synthetic construct
GGVGDDSMA

SEQ ID NO: 38462 - protein, 9 aa, synthetic construct
GGVGDDYMD

SEQ ID NO: 38463 - protein, 9 aa, synthetic construct
GGVGDDWID

SEQ ID NO: 38464 - protein, 9 aa, synthetic construct
GGVGDDWIT

SEQ ID NO: 38465 - protein, 9 aa, synthetic construct
GGVGDDWLD

SEQ ID NO: 38466 - protein, 9 aa, synthetic construct
GGVGDDWLS

SEQ ID NO: 38467 - protein, 9 aa, synthetic construct
GGVGDDWLT

SEQ ID NO: 38468 - protein, 9 aa, synthetic construct
GGVGDDWVV

SEQ ID NO: 38469 - protein, 9 aa, synthetic construct
GGVGDDYID

SEQ ID NO: 38470 - protein, 9 aa, synthetic construct
GGVGDDYIL

SEQ ID NO: 38471 - protein, 9 aa, synthetic construct
GGVGDDYIN

SEQ ID NO: 38472 - protein, 9 aa, synthetic construct
GGVGDDYLA

SEQ ID NO: 38473 - protein, 9 aa, synthetic construct
GGVGDDYLE

SEQ ID NO: 38474 - protein, 9 aa, synthetic construct
GGVGDDYLI

SEQ ID NO: 38475 - protein, 9 aa, synthetic construct
GGVGDDYLW

SEQ ID NO: 38476 - protein, 9 aa, synthetic construct
GGVGDDYMN

SEQ ID NO: 38477 - protein, 9 aa, synthetic construct
GGVGDDVYK

SEQ ID NO: 38478 - protein, 9 aa, synthetic construct
GGVGDDYVS

SEQ ID NO: 38479 - protein, 9 aa, synthetic construct
GGVGEDALF

SEQ ID NO: 38480 - protein, 9 aa, synthetic construct
GGVGEDDLS

SEQ ID NO: 38481 - protein, 9 aa, synthetic construct
GGVGEDDVF

SEQ ID NO: 38482 - protein, 9 aa, synthetic construct
GGVGEDFID

SEQ ID NO: 38483 - protein, 9 aa, synthetic construct
GGVGEDFLS

SEQ ID NO: 38484 - protein, 9 aa, synthetic construct
GGVGEDHLT

SEQ ID NO: 38485 - protein, 9 aa, synthetic construct
GGVGEDIIE

SEQ ID NO: 38486 - protein, 9 aa, synthetic construct
GGVGEDILN

SEQ ID NO: 38487 - protein, 9 aa, synthetic construct
GGVGEDILY

SEQ ID NO: 38488 - protein, 9 aa, synthetic construct
GGVGEDLIF

SEQ ID NO: 38489 - protein, 9 aa, synthetic construct
GGVGEDLIN

SEQ ID NO: 38490 - protein, 9 aa, synthetic construct
GGVGEDLLL

SEQ ID NO: 38491 - protein, 9 aa, synthetic construct
GGVGDDVYY

SEQ ID NO: 38492 - protein, 9 aa, synthetic construct
GGVGDDVVV

SEQ ID NO: 38493 - protein, 9 aa, synthetic construct
GGVGDDSMD

SEQ ID NO: 38494 - protein, 9 aa, synthetic construct
GGVGDDTIR

SEQ ID NO: 38495 - protein, 9 aa, synthetic construct
GGVGDDSMF

SEQ ID NO: 38496 - protein, 9 aa, synthetic construct
GGVGDDSML

SEQ ID NO: 38497 - protein, 9 aa, synthetic construct
GGVGDDSMV

SEQ ID NO: 38498 - protein, 9 aa, synthetic construct
GGVGDDSVD

SEQ ID NO: 38499 - protein, 9 aa, synthetic construct
GGVGDDSYL

SEQ ID NO: 38500 - protein, 9 aa, synthetic construct
GGVGDDSYV

SEQ ID NO: 38501 - protein, 9 aa, synthetic construct
GGVGDDTFF

SEQ ID NO: 38502 - protein, 9 aa, synthetic construct
GGVGDDTFI

SEQ ID NO: 38503 - protein, 9 aa, synthetic construct
GGVGDDTFR

SEQ ID NO: 38504 - protein, 9 aa, synthetic construct
GGVGDDTFY

SEQ ID NO: 38505 - protein, 9 aa, synthetic construct
GGVGDDTIA

SEQ ID NO: 38506 - protein, 9 aa, synthetic construct
GGVGDDTIE

SEQ ID NO: 38507 - protein, 9 aa, synthetic construct
GGVGDDTII

SEQ ID NO: 38508 - protein, 9 aa, synthetic construct
GGVGDDTVN

SEQ ID NO: 38509 - protein, 9 aa, synthetic construct
GGVGDDVVM

SEQ ID NO: 38510 - protein, 9 aa, synthetic construct
GGVGDDTVS

SEQ ID NO: 38511 - protein, 9 aa, synthetic construct
GGVGDDTYE

SEQ ID NO: 38512 - protein, 9 aa, synthetic construct
GGVGDDTYM

SEQ ID NO: 38513 - protein, 9 aa, synthetic construct
GGVGDDVFD

SEQ ID NO: 38514 - protein, 9 aa, synthetic construct
GGVGDDVIE

SEQ ID NO: 38515 - protein, 9 aa, synthetic construct
GGVGDDVIF

SEQ ID NO: 38516 - protein, 9 aa, synthetic construct
GGVGDDVIG

SEQ ID NO: 38517 - protein, 9 aa, synthetic construct
GGVGDDVIT

SEQ ID NO: 38518 - protein, 9 aa, synthetic construct
GGVGDDVIV

SEQ ID NO: 38519 - protein, 9 aa, synthetic construct
GGVGDDVLG

SEQ ID NO: 38520 - protein, 9 aa, synthetic construct
GGVGDDVMN

SEQ ID NO: 38521 - protein, 9 aa, synthetic construct
GGVGDDVVA

SEQ ID NO: 38522 - protein, 9 aa, synthetic construct
GGVGDDVVD

SEQ ID NO: 38523 - protein, 9 aa, synthetic construct
GGVGKDRLL

SEQ ID NO: 38524 - protein, 9 aa, synthetic construct
GGVGKDRMF

SEQ ID NO: 38525 - protein, 9 aa, synthetic construct
GGVGDDKLT

SEQ ID NO: 38526 - protein, 9 aa, synthetic construct
GGVGNDTFD

SEQ ID NO: 38527 - protein, 9 aa, synthetic construct
GGVGNDRIY

SEQ ID NO: 38528 - protein, 9 aa, synthetic construct
GGVGNDRLH

SEQ ID NO: 38529 - protein, 9 aa, synthetic construct
GGVGNDRLW

SEQ ID NO: 38530 - protein, 9 aa, synthetic construct
GGVGNDRMD

SEQ ID NO: 38531 - protein, 9 aa, synthetic construct
GGVGNDRMR

SEQ ID NO: 38532 - protein, 9 aa, synthetic construct
GGVGNDRMS

SEQ ID NO: 38533 - protein, 9 aa, synthetic construct
GGVGNDRVS

SEQ ID NO: 38534 - protein, 9 aa, synthetic construct
GGVGNDRVT

SEQ ID NO: 38535 - protein, 9 aa, synthetic construct
GGVGNDSAI

SEQ ID NO: 38536 - protein, 9 aa, synthetic construct
GGVGNDSIF

SEQ ID NO: 38537 - protein, 9 aa, synthetic construct
GGVGNDSIL

SEQ ID NO: 38538 - protein, 9 aa, synthetic construct
GGVGNDSLG

SEQ ID NO: 38539 - protein, 9 aa, synthetic construct
GGVGNDSLH

SEQ ID NO: 38540 - protein, 9 aa, synthetic construct
GGVGNDSLQ

SEQ ID NO: 38541 - protein, 9 aa, synthetic construct
GGVGNDSMD

SEQ ID NO: 38542 - protein, 9 aa, synthetic construct
GGVGNDSML

SEQ ID NO: 38543 - protein, 9 aa, synthetic construct
GGVGNDSMN

SEQ ID NO: 38544 - protein, 9 aa, synthetic construct
GGVGNDSMT

SEQ ID NO: 38545 - protein, 9 aa, synthetic construct
GGVGNDSVA

SEQ ID NO: 38546 - protein, 9 aa, synthetic construct
GGVGNDSVF

SEQ ID NO: 38547 - protein, 9 aa, synthetic construct
GGVGNDSVS

SEQ ID NO: 38548 - protein, 9 aa, synthetic construct
GGVGNDSVY

SEQ ID NO: 38549 - protein, 9 aa, synthetic construct
GGVGNDSYL

SEQ ID NO: 38550 - protein, 9 aa, synthetic construct
GGVGNDSYV

SEQ ID NO: 38551 - protein, 9 aa, synthetic construct
GGVGNDSYW

SEQ ID NO: 38552 - protein, 9 aa, synthetic construct
GGVGNDTAA

SEQ ID NO: 38553 - protein, 9 aa, synthetic construct
GGVGNDTAG

SEQ ID NO: 38554 - protein, 9 aa, synthetic construct
GGVGNDTAL

SEQ ID NO: 38555 - protein, 9 aa, synthetic construct
GGVGNDTAV

SEQ ID NO: 38556 - protein, 9 aa, synthetic construct
GGVGNDRIW

SEQ ID NO: 38557 - protein, 9 aa, synthetic construct
GGVGNDRIV

SEQ ID NO: 38558 - protein, 9 aa, synthetic construct
GGVGNDRIQ

SEQ ID NO: 38559 - protein, 9 aa, synthetic construct
GGVGNDQLI

SEQ ID NO: 38560 - protein, 9 aa, synthetic construct
GGVGNDNMG

SEQ ID NO: 38561 - protein, 9 aa, synthetic construct
GGVGNDNMN

SEQ ID NO: 38562 - protein, 9 aa, synthetic construct
GGVGNDNMS

SEQ ID NO: 38563 - protein, 9 aa, synthetic construct
GGVGNDNVQ

SEQ ID NO: 38564 - protein, 9 aa, synthetic construct
GGVGNDNYW

SEQ ID NO: 38565 - protein, 9 aa, synthetic construct
GGVGNDQAF

SEQ ID NO: 38566 - protein, 9 aa, synthetic construct
GGVGNDQFV

SEQ ID NO: 38567 - protein, 9 aa, synthetic construct
GGVGNDQIG

SEQ ID NO: 38568 - protein, 9 aa, synthetic construct
GGVGNDQIN

SEQ ID NO: 38569 - protein, 9 aa, synthetic construct
GGVGNDQIT

SEQ ID NO: 38570 - protein, 9 aa, synthetic construct
GGVGNDQIY

SEQ ID NO: 38571 - protein, 9 aa, synthetic construct
GGVGNDQLF

SEQ ID NO: 38572 - protein, 9 aa, synthetic construct
GGVGNDQLH

SEQ ID NO: 38573 - protein, 9 aa, synthetic construct
GGVGNDQLR

SEQ ID NO: 38574 - protein, 9 aa, synthetic construct
GGVGNDRII

SEQ ID NO: 38575 - protein, 9 aa, synthetic construct
GGVGNDQLS

SEQ ID NO: 38576 - protein, 9 aa, synthetic construct
GGVGNDQLV

SEQ ID NO: 38577 - protein, 9 aa, synthetic construct
GGVGNDQMA

SEQ ID NO: 38578 - protein, 9 aa, synthetic construct
GGVGNDQMD

SEQ ID NO: 38579 - protein, 9 aa, synthetic construct
GGVGNDQMT

SEQ ID NO: 38580 - protein, 9 aa, synthetic construct
GGVGNDQVA

SEQ ID NO: 38581 - protein, 9 aa, synthetic construct
GGVGNDQVE

SEQ ID NO: 38582 - protein, 9 aa, synthetic construct
GGVGNDQVF

SEQ ID NO: 38583 - protein, 9 aa, synthetic construct
GGVGNDQVR

SEQ ID NO: 38584 - protein, 9 aa, synthetic construct
GGVGNDQVT

SEQ ID NO: 38585 - protein, 9 aa, synthetic construct
GGVGNDRAN

SEQ ID NO: 38586 - protein, 9 aa, synthetic construct
GGVGNDRAY

SEQ ID NO: 38587 - protein, 9 aa, synthetic construct
GGVGNDRFD

SEQ ID NO: 38588 - protein, 9 aa, synthetic construct
GGVGNDTFA

SEQ ID NO: 38589 - protein, 9 aa, synthetic construct
GGVGNDTIK

SEQ ID NO: 38590 - protein, 9 aa, synthetic construct
GGVGKDSLD

SEQ ID NO: 38591 - protein, 9 aa, synthetic construct
GGVGNDTIM

SEQ ID NO: 38592 - protein, 9 aa, synthetic construct
GGVGNDYID

SEQ ID NO: 38593 - protein, 9 aa, synthetic construct
GGVGNDYIE

SEQ ID NO: 38594 - protein, 9 aa, synthetic construct
GGVGNDYIN

SEQ ID NO: 38595 - protein, 9 aa, synthetic construct
GGVGNDYIY

SEQ ID NO: 38596 - protein, 9 aa, synthetic construct
GGVGNDYLG

SEQ ID NO: 38597 - protein, 9 aa, synthetic construct
GGVGNDYLM

SEQ ID NO: 38598 - protein, 9 aa, synthetic construct
GGVGNDYLT

SEQ ID NO: 38599 - protein, 9 aa, synthetic construct
GGVGNDYVW

SEQ ID NO: 38600 - protein, 9 aa, synthetic construct
GGVGPDMID

SEQ ID NO: 38601 - protein, 9 aa, synthetic construct
GGVGPDRFD

SEQ ID NO: 38602 - protein, 9 aa, synthetic construct
GGVGPDRLA

SEQ ID NO: 38603 - protein, 9 aa, synthetic construct
GGVGPDSLD

SEQ ID NO: 38604 - protein, 9 aa, synthetic construct
GGVGPDSLF

SEQ ID NO: 38605 - protein, 9 aa, synthetic construct
GGVGPDSLT

SEQ ID NO: 38606 - protein, 9 aa, synthetic construct
GGVGPDTLT

SEQ ID NO: 38607 - protein, 9 aa, synthetic construct
GGVGPDVLQ

SEQ ID NO: 38608 - protein, 9 aa, synthetic construct
GGVGQDAIW

SEQ ID NO: 38609 - protein, 9 aa, synthetic construct
GGVGQDEIS

SEQ ID NO: 38610 - protein, 9 aa, synthetic construct
GGVGQDELH

SEQ ID NO: 38611 - protein, 9 aa, synthetic construct
GGVGQDFLA

SEQ ID NO: 38612 - protein, 9 aa, synthetic construct
GGVGQDGIL

SEQ ID NO: 38613 - protein, 9 aa, synthetic construct
GGVGQDIFH

SEQ ID NO: 38614 - protein, 9 aa, synthetic construct
GGVGQDIIF

SEQ ID NO: 38615 - protein, 9 aa, synthetic construct
GGVGQDILL

SEQ ID NO: 38616 - protein, 9 aa, synthetic construct
GGVGQDKLI

SEQ ID NO: 38617 - protein, 9 aa, synthetic construct
GGVGQDLLV

SEQ ID NO: 38618 - protein, 9 aa, synthetic construct
GGVGQDRAF

SEQ ID NO: 38619 - protein, 9 aa, synthetic construct
GGVGQDRLL

SEQ ID NO: 38620 - protein, 9 aa, synthetic construct
GGVGQDRLV

SEQ ID NO: 38621 - protein, 9 aa, synthetic construct
GGVGNDWLK

SEQ ID NO: 38622 - protein, 9 aa, synthetic construct
GGVGNDWLI

SEQ ID NO: 38623 - protein, 9 aa, synthetic construct
GGVGNDWLG

SEQ ID NO: 38624 - protein, 9 aa, synthetic construct
GGVGNDVFN

SEQ ID NO: 38625 - protein, 9 aa, synthetic construct
GGVGNDTIV

SEQ ID NO: 38626 - protein, 9 aa, synthetic construct
GGVGNDTLG

SEQ ID NO: 38627 - protein, 9 aa, synthetic construct
GGVGNDTME

SEQ ID NO: 38628 - protein, 9 aa, synthetic construct
GGVGNDTMY

SEQ ID NO: 38629 - protein, 9 aa, synthetic construct
GGVGNDTVQ

SEQ ID NO: 38630 - protein, 9 aa, synthetic construct
GGVGNDTVS

SEQ ID NO: 38631 - protein, 9 aa, synthetic construct
GGVGNDTVW

SEQ ID NO: 38632 - protein, 9 aa, synthetic construct
GGVGNDTYM

SEQ ID NO: 38633 - protein, 9 aa, synthetic construct
GGVGNDTYS

SEQ ID NO: 38634 - protein, 9 aa, synthetic construct
GGVGNDTYW

SEQ ID NO: 38635 - protein, 9 aa, synthetic construct
GGVGNDVAS

SEQ ID NO: 38636 - protein, 9 aa, synthetic construct
GGVGNDVFD

SEQ ID NO: 38637 - protein, 9 aa, synthetic construct
GGVGNDVFK

SEQ ID NO: 38638 - protein, 9 aa, synthetic construct
GGVGNDVFS

SEQ ID NO: 38639 - protein, 9 aa, synthetic construct
GGVGNDWLE

SEQ ID NO: 38640 - protein, 9 aa, synthetic construct
GGVGNDVIE

SEQ ID NO: 38641 - protein, 9 aa, synthetic construct
GGVGNDVIN

SEQ ID NO: 38642 - protein, 9 aa, synthetic construct
GGVGNDVIY

SEQ ID NO: 38643 - protein, 9 aa, synthetic construct
GGVGNDVLG

SEQ ID NO: 38644 - protein, 9 aa, synthetic construct
GGVGNDVLL

SEQ ID NO: 38645 - protein, 9 aa, synthetic construct
GGVGNDVME

SEQ ID NO: 38646 - protein, 9 aa, synthetic construct
GGVGNDVMS

SEQ ID NO: 38647 - protein, 9 aa, synthetic construct
GGVGNDVMT

SEQ ID NO: 38648 - protein, 9 aa, synthetic construct
GGVGNDVVN

SEQ ID NO: 38649 - protein, 9 aa, synthetic construct
GGVGNDVVR

SEQ ID NO: 38650 - protein, 9 aa, synthetic construct
GGVGNDVVV

SEQ ID NO: 38651 - protein, 9 aa, synthetic construct
GGVGNDVYY

SEQ ID NO: 38652 - protein, 9 aa, synthetic construct
GGVGNDWAF

SEQ ID NO: 38653 - protein, 9 aa, synthetic construct
GGVGNDNLW

SEQ ID NO: 38654 - protein, 9 aa, synthetic construct
GGVGNDNLT

SEQ ID NO: 38655 - protein, 9 aa, synthetic construct
GGVGNDNLS

SEQ ID NO: 38656 - protein, 9 aa, synthetic construct
GGVGNDNLD

SEQ ID NO: 38657 - protein, 9 aa, synthetic construct
GGVGLDTLQ

SEQ ID NO: 38658 - protein, 9 aa, synthetic construct
GGVGLDTLR

SEQ ID NO: 38659 - protein, 9 aa, synthetic construct
GGVGLDTLW

SEQ ID NO: 38660 - protein, 9 aa, synthetic construct
GGVGLDVAI

SEQ ID NO: 38661 - protein, 9 aa, synthetic construct
GGVGLDVLF

SEQ ID NO: 38662 - protein, 9 aa, synthetic construct
GGVGLDVYI

SEQ ID NO: 38663 - protein, 9 aa, synthetic construct
GGVGLDWLL

SEQ ID NO: 38664 - protein, 9 aa, synthetic construct
GGVGMDEFH

SEQ ID NO: 38665 - protein, 9 aa, synthetic construct
GGVGMDELQ

SEQ ID NO: 38666 - protein, 9 aa, synthetic construct
GGVGMDIFA

SEQ ID NO: 38667 - protein, 9 aa, synthetic construct
GGVGMDILT

SEQ ID NO: 38668 - protein, 9 aa, synthetic construct
GGVGMDIMS

SEQ ID NO: 38669 - protein, 9 aa, synthetic construct
GGVGMDRMA

SEQ ID NO: 38670 - protein, 9 aa, synthetic construct
GGVGMDSMS

SEQ ID NO: 38671 - protein, 9 aa, synthetic construct
GGVGMDTLN

SEQ ID NO: 38672 - protein, 9 aa, synthetic construct
GGVGMDTMT

SEQ ID NO: 38673 - protein, 9 aa, synthetic construct
GGVGNDAID

SEQ ID NO: 38674 - protein, 9 aa, synthetic construct
GGVGNDAIN

SEQ ID NO: 38675 - protein, 9 aa, synthetic construct
GGVGNDAIT

SEQ ID NO: 38676 - protein, 9 aa, synthetic construct
GGVGNDALA

SEQ ID NO: 38677 - protein, 9 aa, synthetic construct
GGVGNDALI

SEQ ID NO: 38678 - protein, 9 aa, synthetic construct
GGVGNDALL

SEQ ID NO: 38679 - protein, 9 aa, synthetic construct
GGVGNDALS

SEQ ID NO: 38680 - protein, 9 aa, synthetic construct
GGVGNDALW

SEQ ID NO: 38681 - protein, 9 aa, synthetic construct
GGVGNDAMA

SEQ ID NO: 38682 - protein, 9 aa, synthetic construct
GGVGNDAML

SEQ ID NO: 38683 - protein, 9 aa, synthetic construct
GGVGNDAMR

SEQ ID NO: 38684 - protein, 9 aa, synthetic construct
GGVGNDAMT

SEQ ID NO: 38685 - protein, 9 aa, synthetic construct
GGVGNDDFF

SEQ ID NO: 38686 - protein, 9 aa, synthetic construct
GGVGLDTLI

SEQ ID NO: 38687 - protein, 9 aa, synthetic construct
GGVGLDTLH

SEQ ID NO: 38688 - protein, 9 aa, synthetic construct
GGVGLDTLG

SEQ ID NO: 38689 - protein, 9 aa, synthetic construct
GGVGKDVMF

SEQ ID NO: 38690 - protein, 9 aa, synthetic construct
GGVGKDSLH

SEQ ID NO: 38691 - protein, 9 aa, synthetic construct
GGVGKDSMA

SEQ ID NO: 38692 - protein, 9 aa, synthetic construct
GGVGKDTAQ

SEQ ID NO: 38693 - protein, 9 aa, synthetic construct
GGVGKDTIE

SEQ ID NO: 38694 - protein, 9 aa, synthetic construct
GGVGKDTIL

SEQ ID NO: 38695 - protein, 9 aa, synthetic construct
GGVGKDTIY

SEQ ID NO: 38696 - protein, 9 aa, synthetic construct
GGVGKDTLK

SEQ ID NO: 38697 - protein, 9 aa, synthetic construct
GGVGKDTLN

SEQ ID NO: 38698 - protein, 9 aa, synthetic construct
GGVGKDTLR

SEQ ID NO: 38699 - protein, 9 aa, synthetic construct
GGVGKDTLS

SEQ ID NO: 38700 - protein, 9 aa, synthetic construct
GGVGKDVFN

SEQ ID NO: 38701 - protein, 9 aa, synthetic construct
GGVGKDVFV

SEQ ID NO: 38702 - protein, 9 aa, synthetic construct
GGVGKDVLN

SEQ ID NO: 38703 - protein, 9 aa, synthetic construct
GGVGKDWIS

SEQ ID NO: 38704 - protein, 9 aa, synthetic construct
GGVGLDTLF

SEQ ID NO: 38705 - protein, 9 aa, synthetic construct
GGVGKDWLD

SEQ ID NO: 38706 - protein, 9 aa, synthetic construct
GGVGLDALH

SEQ ID NO: 38707 - protein, 9 aa, synthetic construct
GGVGLDHFR

SEQ ID NO: 38708 - protein, 9 aa, synthetic construct
GGVGLDHLF

SEQ ID NO: 38709 - protein, 9 aa, synthetic construct
GGVGLDQLI

SEQ ID NO: 38710 - protein, 9 aa, synthetic construct
GGVGLDQLW

SEQ ID NO: 38711 - protein, 9 aa, synthetic construct
GGVGLDRAV

SEQ ID NO: 38712 - protein, 9 aa, synthetic construct
GGVGLDRFV

SEQ ID NO: 38713 - protein, 9 aa, synthetic construct
GGVGLDRLE

SEQ ID NO: 38714 - protein, 9 aa, synthetic construct
GGVGLDRLT

SEQ ID NO: 38715 - protein, 9 aa, synthetic construct
GGVGLDSID

SEQ ID NO: 38716 - protein, 9 aa, synthetic construct
GGVGLDSLL

SEQ ID NO: 38717 - protein, 9 aa, synthetic construct
GGVGLDSLW

SEQ ID NO: 38718 - protein, 9 aa, synthetic construct
GGVGNDDIT

SEQ ID NO: 38719 - protein, 9 aa, synthetic construct
GGVGNDDLA

SEQ ID NO: 38720 - protein, 9 aa, synthetic construct
GGVGNDDLE

SEQ ID NO: 38721 - protein, 9 aa, synthetic construct
GGVGNDLIH

SEQ ID NO: 38722 - protein, 9 aa, synthetic construct
GGVGNDIYL

SEQ ID NO: 38723 - protein, 9 aa, synthetic construct
GGVGNDIYY

SEQ ID NO: 38724 - protein, 9 aa, synthetic construct
GGVGNDKAW

SEQ ID NO: 38725 - protein, 9 aa, synthetic construct
GGVGNDKFV

SEQ ID NO: 38726 - protein, 9 aa, synthetic construct
GGVGNDKLI

SEQ ID NO: 38727 - protein, 9 aa, synthetic construct
GGVGNDKLM

SEQ ID NO: 38728 - protein, 9 aa, synthetic construct
GGVGNDKLQ

SEQ ID NO: 38729 - protein, 9 aa, synthetic construct
GGVGNDKLT

SEQ ID NO: 38730 - protein, 9 aa, synthetic construct
GGVGNDKMF

SEQ ID NO: 38731 - protein, 9 aa, synthetic construct
GGVGNDLAD

SEQ ID NO: 38732 - protein, 9 aa, synthetic construct
GGVGNDLAL

SEQ ID NO: 38733 - protein, 9 aa, synthetic construct
GGVGNDLFL

SEQ ID NO: 38734 - protein, 9 aa, synthetic construct
GGVGNDLID

SEQ ID NO: 38735 - protein, 9 aa, synthetic construct
GGVGNDLIL

SEQ ID NO: 38736 - protein, 9 aa, synthetic construct
GGVGNDIVI

SEQ ID NO: 38737 - protein, 9 aa, synthetic construct
GGVGNDLIM

SEQ ID NO: 38738 - protein, 9 aa, synthetic construct
GGVGNDLLG

SEQ ID NO: 38739 - protein, 9 aa, synthetic construct
GGVGNDLLH

SEQ ID NO: 38740 - protein, 9 aa, synthetic construct
GGVGNDLLR

SEQ ID NO: 38741 - protein, 9 aa, synthetic construct
GGVGNDLMD

SEQ ID NO: 38742 - protein, 9 aa, synthetic construct
GGVGNDLVS

SEQ ID NO: 38743 - protein, 9 aa, synthetic construct
GGVGNDLVW

SEQ ID NO: 38744 - protein, 9 aa, synthetic construct
GGVGNDLYF

SEQ ID NO: 38745 - protein, 9 aa, synthetic construct
GGVGNDMLD

SEQ ID NO: 38746 - protein, 9 aa, synthetic construct
GGVGNDMLI

SEQ ID NO: 38747 - protein, 9 aa, synthetic construct
GGVGNDNIA

SEQ ID NO: 38748 - protein, 9 aa, synthetic construct
GGVGNDNIY

SEQ ID NO: 38749 - protein, 9 aa, synthetic construct
GGVGNDNLA

SEQ ID NO: 38750 - protein, 9 aa, synthetic construct
GGVGNDIYE

SEQ ID NO: 38751 - protein, 9 aa, synthetic construct
GGVGNDIMT

SEQ ID NO: 38752 - protein, 9 aa, synthetic construct
GGVGNDDLQ

SEQ ID NO: 38753 - protein, 9 aa, synthetic construct
GGVGNDFVY

SEQ ID NO: 38754 - protein, 9 aa, synthetic construct
GGVGNDDLR

SEQ ID NO: 38755 - protein, 9 aa, synthetic construct
GGVGNDDLS

SEQ ID NO: 38756 - protein, 9 aa, synthetic construct
GGVGNDDLT

SEQ ID NO: 38757 - protein, 9 aa, synthetic construct
GGVGNDDVS

SEQ ID NO: 38758 - protein, 9 aa, synthetic construct
GGVGNDEAY

SEQ ID NO: 38759 - protein, 9 aa, synthetic construct
GGVGNDEIR

SEQ ID NO: 38760 - protein, 9 aa, synthetic construct
GGVGNDEIY

SEQ ID NO: 38761 - protein, 9 aa, synthetic construct
GGVGNDELG

SEQ ID NO: 38762 - protein, 9 aa, synthetic construct
GGVGNDELH

SEQ ID NO: 38763 - protein, 9 aa, synthetic construct
GGVGNDELT

SEQ ID NO: 38764 - protein, 9 aa, synthetic construct
GGVGNDEYT

SEQ ID NO: 38765 - protein, 9 aa, synthetic construct
GGVGNDFID

SEQ ID NO: 38766 - protein, 9 aa, synthetic construct
GGVGNDFIV

SEQ ID NO: 38767 - protein, 9 aa, synthetic construct
GGVGNDGAS

SEQ ID NO: 38768 - protein, 9 aa, synthetic construct
GGVGNDILW

SEQ ID NO: 38769 - protein, 9 aa, synthetic construct
GGVGNDGID

SEQ ID NO: 38770 - protein, 9 aa, synthetic construct
GGVGNDGLT

SEQ ID NO: 38771 - protein, 9 aa, synthetic construct
GGVGNDGYF

SEQ ID NO: 38772 - protein, 9 aa, synthetic construct
GGVGNDHIA

SEQ ID NO: 38773 - protein, 9 aa, synthetic construct
GGVGNDHIY

SEQ ID NO: 38774 - protein, 9 aa, synthetic construct
GGVGNDHLV

SEQ ID NO: 38775 - protein, 9 aa, synthetic construct
GGVGNDHME

SEQ ID NO: 38776 - protein, 9 aa, synthetic construct
GGVGNDIFA

SEQ ID NO: 38777 - protein, 9 aa, synthetic construct
GGVGNDIFN

SEQ ID NO: 38778 - protein, 9 aa, synthetic construct
GGVGNDIIA

SEQ ID NO: 38779 - protein, 9 aa, synthetic construct
GGVGNDIII

SEQ ID NO: 38780 - protein, 9 aa, synthetic construct
GGVGNDILG

SEQ ID NO: 38781 - protein, 9 aa, synthetic construct
GGVGNDILR

SEQ ID NO: 38782 - protein, 9 aa, synthetic construct
GGVGDDKLW

SEQ ID NO: 38783 - protein, 9 aa, synthetic construct
GGVGDDKLQ

SEQ ID NO: 38784 - protein, 9 aa, synthetic construct
GGSGRDLLQ

SEQ ID NO: 38785 - protein, 9 aa, synthetic construct
GGTGTDTVR

SEQ ID NO: 38786 - protein, 9 aa, synthetic construct
GGTGTDSFR

SEQ ID NO: 38787 - protein, 9 aa, synthetic construct
GGTGTDSIA

SEQ ID NO: 38788 - protein, 9 aa, synthetic construct
GGTGTDSIT

SEQ ID NO: 38789 - protein, 9 aa, synthetic construct
GGTGTDSIY

SEQ ID NO: 38790 - protein, 9 aa, synthetic construct
GGTGTDSLA

SEQ ID NO: 38791 - protein, 9 aa, synthetic construct
GGTGTDSLE

SEQ ID NO: 38792 - protein, 9 aa, synthetic construct
GGTGTDSLN

SEQ ID NO: 38793 - protein, 9 aa, synthetic construct
GGTGTDSLT

SEQ ID NO: 38794 - protein, 9 aa, synthetic construct
GGTGTDSMA

SEQ ID NO: 38795 - protein, 9 aa, synthetic construct
GGTGTDSMN

SEQ ID NO: 38796 - protein, 9 aa, synthetic construct
GGTGTDSMS

SEQ ID NO: 38797 - protein, 9 aa, synthetic construct
GGTGTDSVD

SEQ ID NO: 38798 - protein, 9 aa, synthetic construct
GGTGTDSVF

SEQ ID NO: 38799 - protein, 9 aa, synthetic construct
GGTGTDTAG

SEQ ID NO: 38800 - protein, 9 aa, synthetic construct
GGTGTDTAI

SEQ ID NO: 38801 - protein, 9 aa, synthetic construct
GGTGTDTAL

SEQ ID NO: 38802 - protein, 9 aa, synthetic construct
GGTGTDTAM

SEQ ID NO: 38803 - protein, 9 aa, synthetic construct
GGTGTDTAY

SEQ ID NO: 38804 - protein, 9 aa, synthetic construct
GGTGTDTFH

SEQ ID NO: 38805 - protein, 9 aa, synthetic construct
GGTGTDTFL

SEQ ID NO: 38806 - protein, 9 aa, synthetic construct
GGTGTDTFR

SEQ ID NO: 38807 - protein, 9 aa, synthetic construct
GGTGTDTFY

SEQ ID NO: 38808 - protein, 9 aa, synthetic construct
GGTGTDTIA

SEQ ID NO: 38809 - protein, 9 aa, synthetic construct
GGTGTDTIF

SEQ ID NO: 38810 - protein, 9 aa, synthetic construct
GGTGTDTIV

SEQ ID NO: 38811 - protein, 9 aa, synthetic construct
GGTGTDTIY

SEQ ID NO: 38812 - protein, 9 aa, synthetic construct
GGTGTDTLM

SEQ ID NO: 38813 - protein, 9 aa, synthetic construct
GGTGTDTMQ

SEQ ID NO: 38814 - protein, 9 aa, synthetic construct
GGTGTDTMS

SEQ ID NO: 38815 - protein, 9 aa, synthetic construct
GGTGTDSAS

SEQ ID NO: 38816 - protein, 9 aa, synthetic construct
GGTGTDRVY

SEQ ID NO: 38817 - protein, 9 aa, synthetic construct
GGTGTDRML

SEQ ID NO: 38818 - protein, 9 aa, synthetic construct
GGTGTDNFD

SEQ ID NO: 38819 - protein, 9 aa, synthetic construct
GGTGTDILT

SEQ ID NO: 38820 - protein, 9 aa, synthetic construct
GGTGTDILY

SEQ ID NO: 38821 - protein, 9 aa, synthetic construct
GGTGTDKLF

SEQ ID NO: 38822 - protein, 9 aa, synthetic construct
GGTGTDKLI

SEQ ID NO: 38823 - protein, 9 aa, synthetic construct
GGTGTDLAS

SEQ ID NO: 38824 - protein, 9 aa, synthetic construct
GGTGTDLIV

SEQ ID NO: 38825 - protein, 9 aa, synthetic construct
GGTGTDLLE

SEQ ID NO: 38826 - protein, 9 aa, synthetic construct
GGTGTDLLI

SEQ ID NO: 38827 - protein, 9 aa, synthetic construct
GGTGTDLLL

SEQ ID NO: 38828 - protein, 9 aa, synthetic construct
GGTGTDLLY

SEQ ID NO: 38829 - protein, 9 aa, synthetic construct
GGTGTDMAD

SEQ ID NO: 38830 - protein, 9 aa, synthetic construct
GGTGTDMAS

SEQ ID NO: 38831 - protein, 9 aa, synthetic construct
GGTGTDMLY

SEQ ID NO: 38832 - protein, 9 aa, synthetic construct
GGTGTDNIS

SEQ ID NO: 38833 - protein, 9 aa, synthetic construct
GGTGTDRME

SEQ ID NO: 38834 - protein, 9 aa, synthetic construct
GGTGTDNLV

SEQ ID NO: 38835 - protein, 9 aa, synthetic construct
GGTGTDQAN

SEQ ID NO: 38836 - protein, 9 aa, synthetic construct
GGTGTDQIF

SEQ ID NO: 38837 - protein, 9 aa, synthetic construct
GGTGTDQLF

SEQ ID NO: 38838 - protein, 9 aa, synthetic construct
GGTGTDQLI

SEQ ID NO: 38839 - protein, 9 aa, synthetic construct
GGTGTDQMA

SEQ ID NO: 38840 - protein, 9 aa, synthetic construct
GGTGTDQYD

SEQ ID NO: 38841 - protein, 9 aa, synthetic construct
GGTGTDRAF

SEQ ID NO: 38842 - protein, 9 aa, synthetic construct
GGTGTDRIY

SEQ ID NO: 38843 - protein, 9 aa, synthetic construct
GGTGTDRLF

SEQ ID NO: 38844 - protein, 9 aa, synthetic construct
GGTGTDRLN

SEQ ID NO: 38845 - protein, 9 aa, synthetic construct
GGTGTDRLY

SEQ ID NO: 38846 - protein, 9 aa, synthetic construct
GGTGTDRMD

SEQ ID NO: 38847 - protein, 9 aa, synthetic construct
GGTGTDTVA

SEQ ID NO: 38848 - protein, 9 aa, synthetic construct
GGTGTDTVT

SEQ ID NO: 38849 - protein, 9 aa, synthetic construct
GGTGVDSIV

SEQ ID NO: 38850 - protein, 9 aa, synthetic construct
GGTGTDTYV

SEQ ID NO: 38851 - protein, 9 aa, synthetic construct
GGTGVDILT

SEQ ID NO: 38852 - protein, 9 aa, synthetic construct
GGTGVDIML

SEQ ID NO: 38853 - protein, 9 aa, synthetic construct
GGTGVDIMS

SEQ ID NO: 38854 - protein, 9 aa, synthetic construct
GGTGVDIYH

SEQ ID NO: 38855 - protein, 9 aa, synthetic construct
GGTGVDKID

SEQ ID NO: 38856 - protein, 9 aa, synthetic construct
GGTGVDKLI

SEQ ID NO: 38857 - protein, 9 aa, synthetic construct
GGTGVDKLY

SEQ ID NO: 38858 - protein, 9 aa, synthetic construct
GGTGVDKMS

SEQ ID NO: 38859 - protein, 9 aa, synthetic construct
GGTGVDLFV

SEQ ID NO: 38860 - protein, 9 aa, synthetic construct
GGTGVDLID

SEQ ID NO: 38861 - protein, 9 aa, synthetic construct
GGTGVDLII

SEQ ID NO: 38862 - protein, 9 aa, synthetic construct
GGTGVDLLR

SEQ ID NO: 38863 - protein, 9 aa, synthetic construct
GGTGVDLLS

SEQ ID NO: 38864 - protein, 9 aa, synthetic construct
GGTGVDLMN

SEQ ID NO: 38865 - protein, 9 aa, synthetic construct
GGTGVDLMT

SEQ ID NO: 38866 - protein, 9 aa, synthetic construct
GGTGVDLVA

SEQ ID NO: 38867 - protein, 9 aa, synthetic construct
GGTGVDNIF

SEQ ID NO: 38868 - protein, 9 aa, synthetic construct
GGTGVDNLS

SEQ ID NO: 38869 - protein, 9 aa, synthetic construct
GGTGVDQMF

SEQ ID NO: 38870 - protein, 9 aa, synthetic construct
GGTGVDRAQ

SEQ ID NO: 38871 - protein, 9 aa, synthetic construct
GGTGVDRFE

SEQ ID NO: 38872 - protein, 9 aa, synthetic construct
GGTGVDRFR

SEQ ID NO: 38873 - protein, 9 aa, synthetic construct
GGTGVDRFW

SEQ ID NO: 38874 - protein, 9 aa, synthetic construct
GGTGVDRIS

SEQ ID NO: 38875 - protein, 9 aa, synthetic construct
GGTGVDRLS

SEQ ID NO: 38876 - protein, 9 aa, synthetic construct
GGTGVDRMA

SEQ ID NO: 38877 - protein, 9 aa, synthetic construct
GGTGVDRMS

SEQ ID NO: 38878 - protein, 9 aa, synthetic construct
GGTGVDSAF

SEQ ID NO: 38879 - protein, 9 aa, synthetic construct
GGTGVDSIS

SEQ ID NO: 38880 - protein, 9 aa, synthetic construct
GGTGVDILR

SEQ ID NO: 38881 - protein, 9 aa, synthetic construct
GGTGVDILA

SEQ ID NO: 38882 - protein, 9 aa, synthetic construct
GGTGVDIIL

SEQ ID NO: 38883 - protein, 9 aa, synthetic construct
GGTGTDYLF

SEQ ID NO: 38884 - protein, 9 aa, synthetic construct
GGTGTDVAD

SEQ ID NO: 38885 - protein, 9 aa, synthetic construct
GGTGTDVAR

SEQ ID NO: 38886 - protein, 9 aa, synthetic construct
GGTGTDVAY

SEQ ID NO: 38887 - protein, 9 aa, synthetic construct
GGTGTDVFA

SEQ ID NO: 38888 - protein, 9 aa, synthetic construct
GGTGTDVIE

SEQ ID NO: 38889 - protein, 9 aa, synthetic construct
GGTGTDVLL

SEQ ID NO: 38890 - protein, 9 aa, synthetic construct
GGTGTDVLR

SEQ ID NO: 38891 - protein, 9 aa, synthetic construct
GGTGTDVMI

SEQ ID NO: 38892 - protein, 9 aa, synthetic construct
GGTGTDVYF

SEQ ID NO: 38893 - protein, 9 aa, synthetic construct
GGTGTDWLA

SEQ ID NO: 38894 - protein, 9 aa, synthetic construct
GGTGTDYFI

SEQ ID NO: 38895 - protein, 9 aa, synthetic construct
GGTGTDYID

SEQ ID NO: 38896 - protein, 9 aa, synthetic construct
GGTGTDYLE

SEQ ID NO: 38897 - protein, 9 aa, synthetic construct
GGTGTDYVS

SEQ ID NO: 38898 - protein, 9 aa, synthetic construct
GGTGVDIFR

SEQ ID NO: 38899 - protein, 9 aa, synthetic construct
GGTGTDYVW

SEQ ID NO: 38900 - protein, 9 aa, synthetic construct
GGTGVDALT

SEQ ID NO: 38901 - protein, 9 aa, synthetic construct
GGTGVDAMA

SEQ ID NO: 38902 - protein, 9 aa, synthetic construct
GGTGVDDLS

SEQ ID NO: 38903 - protein, 9 aa, synthetic construct
GGTGVDDLY

SEQ ID NO: 38904 - protein, 9 aa, synthetic construct
GGTGVDEFF

SEQ ID NO: 38905 - protein, 9 aa, synthetic construct
GGTGVDELS

SEQ ID NO: 38906 - protein, 9 aa, synthetic construct
GGTGVDFID

SEQ ID NO: 38907 - protein, 9 aa, synthetic construct
GGTGVDFLE

SEQ ID NO: 38908 - protein, 9 aa, synthetic construct
GGTGVDFMI

SEQ ID NO: 38909 - protein, 9 aa, synthetic construct
GGTGVDGVV

SEQ ID NO: 38910 - protein, 9 aa, synthetic construct
GGTGVDHLE

SEQ ID NO: 38911 - protein, 9 aa, synthetic construct
GGTGVDHLL

SEQ ID NO: 38912 - protein, 9 aa, synthetic construct
GGTGTDILS

SEQ ID NO: 38913 - protein, 9 aa, synthetic construct
GGTGTDIIL

SEQ ID NO: 38914 - protein, 9 aa, synthetic construct
GGTGTDIID

SEQ ID NO: 38915 - protein, 9 aa, synthetic construct
GGTGTDIFV

SEQ ID NO: 38916 - protein, 9 aa, synthetic construct
GGTGSDQMS

SEQ ID NO: 38917 - protein, 9 aa, synthetic construct
GGTGSDRAM

SEQ ID NO: 38918 - protein, 9 aa, synthetic construct
GGTGSDRFD

SEQ ID NO: 38919 - protein, 9 aa, synthetic construct
GGTGSDRFF

SEQ ID NO: 38920 - protein, 9 aa, synthetic construct
GGTGSDRIY

SEQ ID NO: 38921 - protein, 9 aa, synthetic construct
GGTGSDRLF

SEQ ID NO: 38922 - protein, 9 aa, synthetic construct
GGTGSDRLQ

SEQ ID NO: 38923 - protein, 9 aa, synthetic construct
GGTGSDRVF

SEQ ID NO: 38924 - protein, 9 aa, synthetic construct
GGTGSDSII

SEQ ID NO: 38925 - protein, 9 aa, synthetic construct
GGTGSDSIS

SEQ ID NO: 38926 - protein, 9 aa, synthetic construct
GGTGSDSIT

SEQ ID NO: 38927 - protein, 9 aa, synthetic construct
GGTGSDSIY

SEQ ID NO: 38928 - protein, 9 aa, synthetic construct
GGTGSDSLH

SEQ ID NO: 38929 - protein, 9 aa, synthetic construct
GGTGSDSLK

SEQ ID NO: 38930 - protein, 9 aa, synthetic construct
GGTGSDSLW

SEQ ID NO: 38931 - protein, 9 aa, synthetic construct
GGTGSDSMA

SEQ ID NO: 38932 - protein, 9 aa, synthetic construct
GGTGSDSMF

SEQ ID NO: 38933 - protein, 9 aa, synthetic construct
GGTGSDSMI

SEQ ID NO: 38934 - protein, 9 aa, synthetic construct
GGTGSDSYV

SEQ ID NO: 38935 - protein, 9 aa, synthetic construct
GGTGSDTAM

SEQ ID NO: 38936 - protein, 9 aa, synthetic construct
GGTGSDTAY

SEQ ID NO: 38937 - protein, 9 aa, synthetic construct
GGTGSDTFA

SEQ ID NO: 38938 - protein, 9 aa, synthetic construct
GGTGSDTFI

SEQ ID NO: 38939 - protein, 9 aa, synthetic construct
GGTGSDTIF

SEQ ID NO: 38940 - protein, 9 aa, synthetic construct
GGTGSDTIK

SEQ ID NO: 38941 - protein, 9 aa, synthetic construct
GGTGSDTIN

SEQ ID NO: 38942 - protein, 9 aa, synthetic construct
GGTGSDTIR

SEQ ID NO: 38943 - protein, 9 aa, synthetic construct
GGTGSDTIY

SEQ ID NO: 38944 - protein, 9 aa, synthetic construct
GGTGSDTLM

SEQ ID NO: 38945 - protein, 9 aa, synthetic construct
GGTGSDQLW

SEQ ID NO: 38946 - protein, 9 aa, synthetic construct
GGTGSDQLQ

SEQ ID NO: 38947 - protein, 9 aa, synthetic construct
GGTGSDQIW

SEQ ID NO: 38948 - protein, 9 aa, synthetic construct
GGTGSDLVY

SEQ ID NO: 38949 - protein, 9 aa, synthetic construct
GGTGSDKLA

SEQ ID NO: 38950 - protein, 9 aa, synthetic construct
GGTGSDKLQ

SEQ ID NO: 38951 - protein, 9 aa, synthetic construct
GGTGSDLFR

SEQ ID NO: 38952 - protein, 9 aa, synthetic construct
GGTGSDLIF

SEQ ID NO: 38953 - protein, 9 aa, synthetic construct
GGTGSDLIH

SEQ ID NO: 38954 - protein, 9 aa, synthetic construct
GGTGSDLIN

SEQ ID NO: 38955 - protein, 9 aa, synthetic construct
GGTGSDLIQ

SEQ ID NO: 38956 - protein, 9 aa, synthetic construct
GGTGSDLLH

SEQ ID NO: 38957 - protein, 9 aa, synthetic construct
GGTGSDLLM

SEQ ID NO: 38958 - protein, 9 aa, synthetic construct
GGTGSDLLV

SEQ ID NO: 38959 - protein, 9 aa, synthetic construct
GGTGSDLLW

SEQ ID NO: 38960 - protein, 9 aa, synthetic construct
GGTGSDLVR

SEQ ID NO: 38961 - protein, 9 aa, synthetic construct
GGTGSDLVS

SEQ ID NO: 38962 - protein, 9 aa, synthetic construct
GGTGSDLYY

SEQ ID NO: 38963 - protein, 9 aa, synthetic construct
GGTGSDQIR

SEQ ID NO: 38964 - protein, 9 aa, synthetic construct
GGTGSDMFI

SEQ ID NO: 38965 - protein, 9 aa, synthetic construct
GGTGSDMFV

SEQ ID NO: 38966 - protein, 9 aa, synthetic construct
GGTGSDMID

SEQ ID NO: 38967 - protein, 9 aa, synthetic construct
GGTGSDMIY

SEQ ID NO: 38968 - protein, 9 aa, synthetic construct
GGTGSDMLT

SEQ ID NO: 38969 - protein, 9 aa, synthetic construct
GGTGSDMYR

SEQ ID NO: 38970 - protein, 9 aa, synthetic construct
GGTGSDNFL

SEQ ID NO: 38971 - protein, 9 aa, synthetic construct
GGTGSDNID

SEQ ID NO: 38972 - protein, 9 aa, synthetic construct
GGTGSDNIF

SEQ ID NO: 38973 - protein, 9 aa, synthetic construct
GGTGSDNMK

SEQ ID NO: 38974 - protein, 9 aa, synthetic construct
GGTGSDQFK

SEQ ID NO: 38975 - protein, 9 aa, synthetic construct
GGTGSDQFL

SEQ ID NO: 38976 - protein, 9 aa, synthetic construct
GGTGSDQIQ

SEQ ID NO: 38977 - protein, 9 aa, synthetic construct
GGTGSDTLW

SEQ ID NO: 38978 - protein, 9 aa, synthetic construct
GGTGSDTMF

SEQ ID NO: 38979 - protein, 9 aa, synthetic construct
GGTGSDTMG

SEQ ID NO: 38980 - protein, 9 aa, synthetic construct
GGTGTDAMI

SEQ ID NO: 38981 - protein, 9 aa, synthetic construct
GGTGSDYFI

SEQ ID NO: 38982 - protein, 9 aa, synthetic construct
GGTGSDYFV

SEQ ID NO: 38983 - protein, 9 aa, synthetic construct
GGTGSDYIE

SEQ ID NO: 38984 - protein, 9 aa, synthetic construct
GGTGSDYIL

SEQ ID NO: 38985 - protein, 9 aa, synthetic construct
GGTGSDYLH

SEQ ID NO: 38986 - protein, 9 aa, synthetic construct
GGTGSDYLI

SEQ ID NO: 38987 - protein, 9 aa, synthetic construct
GGTGSDYMK

SEQ ID NO: 38988 - protein, 9 aa, synthetic construct
GGTGSDYMT

SEQ ID NO: 38989 - protein, 9 aa, synthetic construct
GGTGSDYVN

SEQ ID NO: 38990 - protein, 9 aa, synthetic construct
GGTGSDYVT

SEQ ID NO: 38991 - protein, 9 aa, synthetic construct
GGTGTDAAD

SEQ ID NO: 38992 - protein, 9 aa, synthetic construct
GGTGTDAAS

SEQ ID NO: 38993 - protein, 9 aa, synthetic construct
GGTGTDALR

SEQ ID NO: 38994 - protein, 9 aa, synthetic construct
GGTGTDCIY

SEQ ID NO: 38995 - protein, 9 aa, synthetic construct
GGTGSDWMV

SEQ ID NO: 38996 - protein, 9 aa, synthetic construct
GGTGTDELY

SEQ ID NO: 38997 - protein, 9 aa, synthetic construct
GGTGTDEMI

SEQ ID NO: 38998 - protein, 9 aa, synthetic construct
GGTGTDFLN

SEQ ID NO: 38999 - protein, 9 aa, synthetic construct
GGTGTDFLR

SEQ ID NO: 39000 - protein, 9 aa, synthetic construct
GGTGTDFLS

SEQ ID NO: 39001 - protein, 9 aa, synthetic construct
GGTGTDFMD

SEQ ID NO: 39002 - protein, 9 aa, synthetic construct
GGTGTDFVI

SEQ ID NO: 39003 - protein, 9 aa, synthetic construct
GGTGTDGFR

SEQ ID NO: 39004 - protein, 9 aa, synthetic construct
GGTGTDGLT

SEQ ID NO: 39005 - protein, 9 aa, synthetic construct
GGTGTDGVI

SEQ ID NO: 39006 - protein, 9 aa, synthetic construct
GGTGTDHLS

SEQ ID NO: 39007 - protein, 9 aa, synthetic construct
GGTGTDHLY

SEQ ID NO: 39008 - protein, 9 aa, synthetic construct
GGTGTDIAA

SEQ ID NO: 39009 - protein, 9 aa, synthetic construct
GGTGSDYAS

SEQ ID NO: 39010 - protein, 9 aa, synthetic construct
GGTGSDWLE

SEQ ID NO: 39011 - protein, 9 aa, synthetic construct
GGTGSDTML

SEQ ID NO: 39012 - protein, 9 aa, synthetic construct
GGTGSDVFK

SEQ ID NO: 39013 - protein, 9 aa, synthetic construct
GGTGSDTVD

SEQ ID NO: 39014 - protein, 9 aa, synthetic construct
GGTGSDTVF

SEQ ID NO: 39015 - protein, 9 aa, synthetic construct
GGTGSDTVG

SEQ ID NO: 39016 - protein, 9 aa, synthetic construct
GGTGSDTVK

SEQ ID NO: 39017 - protein, 9 aa, synthetic construct
GGTGSDTVN

SEQ ID NO: 39018 - protein, 9 aa, synthetic construct
GGTGSDTYA

SEQ ID NO: 39019 - protein, 9 aa, synthetic construct
GGTGSDTYM

SEQ ID NO: 39020 - protein, 9 aa, synthetic construct
GGTGSDTYN

SEQ ID NO: 39021 - protein, 9 aa, synthetic construct
GGTGSDTYS

SEQ ID NO: 39022 - protein, 9 aa, synthetic construct
GGTGSDTYW

SEQ ID NO: 39023 - protein, 9 aa, synthetic construct
GGTGSDVAD

SEQ ID NO: 39024 - protein, 9 aa, synthetic construct
GGTGSDVAI

SEQ ID NO: 39025 - protein, 9 aa, synthetic construct
GGTGSDVFF

SEQ ID NO: 39026 - protein, 9 aa, synthetic construct
GGTGSDVIA

SEQ ID NO: 39027 - protein, 9 aa, synthetic construct
GGTGSDWIH

SEQ ID NO: 39028 - protein, 9 aa, synthetic construct
GGTGSDVIK

SEQ ID NO: 39029 - protein, 9 aa, synthetic construct
GGTGSDVIL

SEQ ID NO: 39030 - protein, 9 aa, synthetic construct
GGTGSDVLK

SEQ ID NO: 39031 - protein, 9 aa, synthetic construct
GGTGSDVLY

SEQ ID NO: 39032 - protein, 9 aa, synthetic construct
GGTGSDVMF

SEQ ID NO: 39033 - protein, 9 aa, synthetic construct
GGTGSDVMQ

SEQ ID NO: 39034 - protein, 9 aa, synthetic construct
GGTGSDVMR

SEQ ID NO: 39035 - protein, 9 aa, synthetic construct
GGTGSDVVE

SEQ ID NO: 39036 - protein, 9 aa, synthetic construct
GGTGSDVVF

SEQ ID NO: 39037 - protein, 9 aa, synthetic construct
GGTGSDVVH

SEQ ID NO: 39038 - protein, 9 aa, synthetic construct
GGTGSDVYH

SEQ ID NO: 39039 - protein, 9 aa, synthetic construct
GGTGSDVYL

SEQ ID NO: 39040 - protein, 9 aa, synthetic construct
GGTGSDVYY

SEQ ID NO: 39041 - protein, 9 aa, synthetic construct
GGTGVDSIT

SEQ ID NO: 39042 - protein, 9 aa, synthetic construct
GGTGVDSLD

SEQ ID NO: 39043 - protein, 9 aa, synthetic construct
GGVGDDKLL

SEQ ID NO: 39044 - protein, 9 aa, synthetic construct
GGVGADVMS

SEQ ID NO: 39045 - protein, 9 aa, synthetic construct
GGVGADSIS

SEQ ID NO: 39046 - protein, 9 aa, synthetic construct
GGVGADSLN

SEQ ID NO: 39047 - protein, 9 aa, synthetic construct
GGVGADSLW

SEQ ID NO: 39048 - protein, 9 aa, synthetic construct
GGVGADSMD

SEQ ID NO: 39049 - protein, 9 aa, synthetic construct
GGVGADSMY

SEQ ID NO: 39050 - protein, 9 aa, synthetic construct
GGVGADSVD

SEQ ID NO: 39051 - protein, 9 aa, synthetic construct
GGVGADSVI

SEQ ID NO: 39052 - protein, 9 aa, synthetic construct
GGVGADSVL

SEQ ID NO: 39053 - protein, 9 aa, synthetic construct
GGVGADSVV

SEQ ID NO: 39054 - protein, 9 aa, synthetic construct
GGVGADTFE

SEQ ID NO: 39055 - protein, 9 aa, synthetic construct
GGVGADTFL

SEQ ID NO: 39056 - protein, 9 aa, synthetic construct
GGVGADTIF

SEQ ID NO: 39057 - protein, 9 aa, synthetic construct
GGVGADTLA

SEQ ID NO: 39058 - protein, 9 aa, synthetic construct
GGVGADTLF

SEQ ID NO: 39059 - protein, 9 aa, synthetic construct
GGVGADTLH

SEQ ID NO: 39060 - protein, 9 aa, synthetic construct
GGVGADTME

SEQ ID NO: 39061 - protein, 9 aa, synthetic construct
GGVGADTMK

SEQ ID NO: 39062 - protein, 9 aa, synthetic construct
GGVGADTMN

SEQ ID NO: 39063 - protein, 9 aa, synthetic construct
GGVGADTMS

SEQ ID NO: 39064 - protein, 9 aa, synthetic construct
GGVGADTMV

SEQ ID NO: 39065 - protein, 9 aa, synthetic construct
GGVGADVAH

SEQ ID NO: 39066 - protein, 9 aa, synthetic construct
GGVGADVFA

SEQ ID NO: 39067 - protein, 9 aa, synthetic construct
GGVGADVFQ

SEQ ID NO: 39068 - protein, 9 aa, synthetic construct
GGVGADVFS

SEQ ID NO: 39069 - protein, 9 aa, synthetic construct
GGVGADVIA

SEQ ID NO: 39070 - protein, 9 aa, synthetic construct
GGVGADVIG

SEQ ID NO: 39071 - protein, 9 aa, synthetic construct
GGVGADVLA

SEQ ID NO: 39072 - protein, 9 aa, synthetic construct
GGVGADVLK

SEQ ID NO: 39073 - protein, 9 aa, synthetic construct
GGVGADVLQ

SEQ ID NO: 39074 - protein, 9 aa, synthetic construct
GGVGADSIN

SEQ ID NO: 39075 - protein, 9 aa, synthetic construct
GGVGADSIL

SEQ ID NO: 39076 - protein, 9 aa, synthetic construct
GGVGADSFF

SEQ ID NO: 39077 - protein, 9 aa, synthetic construct
GGVGADMLF

SEQ ID NO: 39078 - protein, 9 aa, synthetic construct
GGVGADLIL

SEQ ID NO: 39079 - protein, 9 aa, synthetic construct
GGVGADLLF

SEQ ID NO: 39080 - protein, 9 aa, synthetic construct
GGVGADLLH

SEQ ID NO: 39081 - protein, 9 aa, synthetic construct
GGVGADLLL

SEQ ID NO: 39082 - protein, 9 aa, synthetic construct
GGVGADLLQ

SEQ ID NO: 39083 - protein, 9 aa, synthetic construct
GGVGADLLR

SEQ ID NO: 39084 - protein, 9 aa, synthetic construct
GGVGADLLS

SEQ ID NO: 39085 - protein, 9 aa, synthetic construct
GGVGADLLV

SEQ ID NO: 39086 - protein, 9 aa, synthetic construct
GGVGADLMA

SEQ ID NO: 39087 - protein, 9 aa, synthetic construct
GGVGADLME

SEQ ID NO: 39088 - protein, 9 aa, synthetic construct
GGVGADLMK

SEQ ID NO: 39089 - protein, 9 aa, synthetic construct
GGVGADLMQ

SEQ ID NO: 39090 - protein, 9 aa, synthetic construct
GGVGADLVS

SEQ ID NO: 39091 - protein, 9 aa, synthetic construct
GGVGADMLQ

SEQ ID NO: 39092 - protein, 9 aa, synthetic construct
GGVGADRVV

SEQ ID NO: 39093 - protein, 9 aa, synthetic construct
GGVGADMLS

SEQ ID NO: 39094 - protein, 9 aa, synthetic construct
GGVGADNIS

SEQ ID NO: 39095 - protein, 9 aa, synthetic construct
GGVGADNLF

SEQ ID NO: 39096 - protein, 9 aa, synthetic construct
GGVGADNVR

SEQ ID NO: 39097 - protein, 9 aa, synthetic construct
GGVGADQFI

SEQ ID NO: 39098 - protein, 9 aa, synthetic construct
GGVGADQFR

SEQ ID NO: 39099 - protein, 9 aa, synthetic construct
GGVGADQLA

SEQ ID NO: 39100 - protein, 9 aa, synthetic construct
GGVGADQLD

SEQ ID NO: 39101 - protein, 9 aa, synthetic construct
GGVGADQLQ

SEQ ID NO: 39102 - protein, 9 aa, synthetic construct
GGVGADQLS

SEQ ID NO: 39103 - protein, 9 aa, synthetic construct
GGVGADRIW

SEQ ID NO: 39104 - protein, 9 aa, synthetic construct
GGVGADRLK

SEQ ID NO: 39105 - protein, 9 aa, synthetic construct
GGVGADRMN

SEQ ID NO: 39106 - protein, 9 aa, synthetic construct
GGVGADVLR

SEQ ID NO: 39107 - protein, 9 aa, synthetic construct
GGVGADVVS

SEQ ID NO: 39108 - protein, 9 aa, synthetic construct
GGTGVDSLN

SEQ ID NO: 39109 - protein, 9 aa, synthetic construct
GGVGADVVT

SEQ ID NO: 39110 - protein, 9 aa, synthetic construct
GGVGDDEVA

SEQ ID NO: 39111 - protein, 9 aa, synthetic construct
GGVGDDFFS

SEQ ID NO: 39112 - protein, 9 aa, synthetic construct
GGVGDDFIQ

SEQ ID NO: 39113 - protein, 9 aa, synthetic construct
GGVGDDFIS

SEQ ID NO: 39114 - protein, 9 aa, synthetic construct
GGVGDDFLF

SEQ ID NO: 39115 - protein, 9 aa, synthetic construct
GGVGDDFLQ

SEQ ID NO: 39116 - protein, 9 aa, synthetic construct
GGVGDDFLT

SEQ ID NO: 39117 - protein, 9 aa, synthetic construct
GGVGDDFLV

SEQ ID NO: 39118 - protein, 9 aa, synthetic construct
GGVGDDFMA

SEQ ID NO: 39119 - protein, 9 aa, synthetic construct
GGVGDDFVQ

SEQ ID NO: 39120 - protein, 9 aa, synthetic construct
GGVGDDGVF

SEQ ID NO: 39121 - protein, 9 aa, synthetic construct
GGVGDDHLE

SEQ ID NO: 39122 - protein, 9 aa, synthetic construct
GGVGDDHLN

SEQ ID NO: 39123 - protein, 9 aa, synthetic construct
GGVGDDHLQ

SEQ ID NO: 39124 - protein, 9 aa, synthetic construct
GGVGDDHLT

SEQ ID NO: 39125 - protein, 9 aa, synthetic construct
GGVGDDIAI

SEQ ID NO: 39126 - protein, 9 aa, synthetic construct
GGVGDDIFS

SEQ ID NO: 39127 - protein, 9 aa, synthetic construct
GGVGDDIFV

SEQ ID NO: 39128 - protein, 9 aa, synthetic construct
GGVGDDIIS

SEQ ID NO: 39129 - protein, 9 aa, synthetic construct
GGVGDDILE

SEQ ID NO: 39130 - protein, 9 aa, synthetic construct
GGVGDDILG

SEQ ID NO: 39131 - protein, 9 aa, synthetic construct
GGVGDDILH

SEQ ID NO: 39132 - protein, 9 aa, synthetic construct
GGVGDDILK

SEQ ID NO: 39133 - protein, 9 aa, synthetic construct
GGVGDDILW

SEQ ID NO: 39134 - protein, 9 aa, synthetic construct
GGVGDDIVR

SEQ ID NO: 39135 - protein, 9 aa, synthetic construct
GGVGDDIYA

SEQ ID NO: 39136 - protein, 9 aa, synthetic construct
GGVGDDKIA

SEQ ID NO: 39137 - protein, 9 aa, synthetic construct
GGVGDDKIY

SEQ ID NO: 39138 - protein, 9 aa, synthetic construct
GGVGDDKLK

SEQ ID NO: 39139 - protein, 9 aa, synthetic construct
GGVGDDELH

SEQ ID NO: 39140 - protein, 9 aa, synthetic construct
GGVGDDELF

SEQ ID NO: 39141 - protein, 9 aa, synthetic construct
GGVGDDEIV

SEQ ID NO: 39142 - protein, 9 aa, synthetic construct
GGVGDDALF

SEQ ID NO: 39143 - protein, 9 aa, synthetic construct
GGVGADVYL

SEQ ID NO: 39144 - protein, 9 aa, synthetic construct
GGVGADVYR

SEQ ID NO: 39145 - protein, 9 aa, synthetic construct
GGVGADWLI

SEQ ID NO: 39146 - protein, 9 aa, synthetic construct
GGVGADWVV

SEQ ID NO: 39147 - protein, 9 aa, synthetic construct
GGVGADYFY

SEQ ID NO: 39148 - protein, 9 aa, synthetic construct
GGVGADYLD

SEQ ID NO: 39149 - protein, 9 aa, synthetic construct
GGVGADYLN

SEQ ID NO: 39150 - protein, 9 aa, synthetic construct
GGVGADYLV

SEQ ID NO: 39151 - protein, 9 aa, synthetic construct
GGVGADYVT

SEQ ID NO: 39152 - protein, 9 aa, synthetic construct
GGVGCDILV

SEQ ID NO: 39153 - protein, 9 aa, synthetic construct
GGVGCDVLI

SEQ ID NO: 39154 - protein, 9 aa, synthetic construct
GGVGCDVLR

SEQ ID NO: 39155 - protein, 9 aa, synthetic construct
GGVGCDVLV

SEQ ID NO: 39156 - protein, 9 aa, synthetic construct
GGVGDDALH

SEQ ID NO: 39157 - protein, 9 aa, synthetic construct
GGVGDDEII

SEQ ID NO: 39158 - protein, 9 aa, synthetic construct
GGVGDDALK

SEQ ID NO: 39159 - protein, 9 aa, synthetic construct
GGVGDDALN

SEQ ID NO: 39160 - protein, 9 aa, synthetic construct
GGVGDDALQ

SEQ ID NO: 39161 - protein, 9 aa, synthetic construct
GGVGDDALS

SEQ ID NO: 39162 - protein, 9 aa, synthetic construct
GGVGDDALY

SEQ ID NO: 39163 - protein, 9 aa, synthetic construct
GGVGDDCLF

SEQ ID NO: 39164 - protein, 9 aa, synthetic construct
GGVGDDDID

SEQ ID NO: 39165 - protein, 9 aa, synthetic construct
GGVGDDDIR

SEQ ID NO: 39166 - protein, 9 aa, synthetic construct
GGVGDDDLD

SEQ ID NO: 39167 - protein, 9 aa, synthetic construct
GGVGDDDLN

SEQ ID NO: 39168 - protein, 9 aa, synthetic construct
GGVGDDDLQ

SEQ ID NO: 39169 - protein, 9 aa, synthetic construct
GGVGDDDMN

SEQ ID NO: 39170 - protein, 9 aa, synthetic construct
GGVGDDEID

SEQ ID NO: 39171 - protein, 9 aa, synthetic construct
GGVGADLIF

SEQ ID NO: 39172 - protein, 9 aa, synthetic construct
GGVGADLID

SEQ ID NO: 39173 - protein, 9 aa, synthetic construct
GGVGADLIA

SEQ ID NO: 39174 - protein, 9 aa, synthetic construct
GGVGADLFL

SEQ ID NO: 39175 - protein, 9 aa, synthetic construct
GGTGVDVVY

SEQ ID NO: 39176 - protein, 9 aa, synthetic construct
GGTGVDWLV

SEQ ID NO: 39177 - protein, 9 aa, synthetic construct
GGTGVDYIE

SEQ ID NO: 39178 - protein, 9 aa, synthetic construct
GGTGVDYLN

SEQ ID NO: 39179 - protein, 9 aa, synthetic construct
GGTGVDYLV

SEQ ID NO: 39180 - protein, 9 aa, synthetic construct
GGTGVDYLY

SEQ ID NO: 39181 - protein, 9 aa, synthetic construct
GGTGVDYMV

SEQ ID NO: 39182 - protein, 9 aa, synthetic construct
GGTGVDYVD

SEQ ID NO: 39183 - protein, 9 aa, synthetic construct
GGTGWDHIY

SEQ ID NO: 39184 - protein, 9 aa, synthetic construct
GGTGWDNVN

SEQ ID NO: 39185 - protein, 9 aa, synthetic construct
GGTGWDRLE

SEQ ID NO: 39186 - protein, 9 aa, synthetic construct
GGTGWDTLD

SEQ ID NO: 39187 - protein, 9 aa, synthetic construct
GGTGXDLLA

SEQ ID NO: 39188 - protein, 9 aa, synthetic construct
GGTGYDCVA

SEQ ID NO: 39189 - protein, 9 aa, synthetic construct
GGTGYDDMY

SEQ ID NO: 39190 - protein, 9 aa, synthetic construct
GGTGYDEMY

SEQ ID NO: 39191 - protein, 9 aa, synthetic construct
GGTGYDFIA

SEQ ID NO: 39192 - protein, 9 aa, synthetic construct
GGTGYDIFE

SEQ ID NO: 39193 - protein, 9 aa, synthetic construct
GGTGYDILF

SEQ ID NO: 39194 - protein, 9 aa, synthetic construct
GGTGYDILI

SEQ ID NO: 39195 - protein, 9 aa, synthetic construct
GGTGYDILT

SEQ ID NO: 39196 - protein, 9 aa, synthetic construct
GGTGYDKLH

SEQ ID NO: 39197 - protein, 9 aa, synthetic construct
GGTGYDLIT

SEQ ID NO: 39198 - protein, 9 aa, synthetic construct
GGTGYDLLA

SEQ ID NO: 39199 - protein, 9 aa, synthetic construct
GGTGYDLLI

SEQ ID NO: 39200 - protein, 9 aa, synthetic construct
GGTGYDLMY

SEQ ID NO: 39201 - protein, 9 aa, synthetic construct
GGTGYDQLD

SEQ ID NO: 39202 - protein, 9 aa, synthetic construct
GGTGYDQLI

SEQ ID NO: 39203 - protein, 9 aa, synthetic construct
GGTGYDRIW

SEQ ID NO: 39204 - protein, 9 aa, synthetic construct
GGTGVDVVH

SEQ ID NO: 39205 - protein, 9 aa, synthetic construct
GGTGVDVMY

SEQ ID NO: 39206 - protein, 9 aa, synthetic construct
GGTGVDVMV

SEQ ID NO: 39207 - protein, 9 aa, synthetic construct
GGTGVDTLA

SEQ ID NO: 39208 - protein, 9 aa, synthetic construct
GGTGVDSLS

SEQ ID NO: 39209 - protein, 9 aa, synthetic construct
GGTGVDSME

SEQ ID NO: 39210 - protein, 9 aa, synthetic construct
GGTGVDSML

SEQ ID NO: 39211 - protein, 9 aa, synthetic construct
GGTGVDSVD

SEQ ID NO: 39212 - protein, 9 aa, synthetic construct
GGTGVDSYR

SEQ ID NO: 39213 - protein, 9 aa, synthetic construct
GGTGVDTAD

SEQ ID NO: 39214 - protein, 9 aa, synthetic construct
GGTGVDTAY

SEQ ID NO: 39215 - protein, 9 aa, synthetic construct
GGTGVDTFG

SEQ ID NO: 39216 - protein, 9 aa, synthetic construct
GGTGVDTFI

SEQ ID NO: 39217 - protein, 9 aa, synthetic construct
GGTGVDTFL

SEQ ID NO: 39218 - protein, 9 aa, synthetic construct
GGTGVDTFT

SEQ ID NO: 39219 - protein, 9 aa, synthetic construct
GGTGVDTID

SEQ ID NO: 39220 - protein, 9 aa, synthetic construct
GGTGVDTIV

SEQ ID NO: 39221 - protein, 9 aa, synthetic construct
GGTGVDTLE

SEQ ID NO: 39222 - protein, 9 aa, synthetic construct
GGTGVDVMQ

SEQ ID NO: 39223 - protein, 9 aa, synthetic construct
GGTGVDTLR

SEQ ID NO: 39224 - protein, 9 aa, synthetic construct
GGTGVDTMR

SEQ ID NO: 39225 - protein, 9 aa, synthetic construct
GGTGVDTVL

SEQ ID NO: 39226 - protein, 9 aa, synthetic construct
GGTGVDTVS

SEQ ID NO: 39227 - protein, 9 aa, synthetic construct
GGTGVDTYY

SEQ ID NO: 39228 - protein, 9 aa, synthetic construct
GGTGVDVAQ

SEQ ID NO: 39229 - protein, 9 aa, synthetic construct
GGTGVDVFV

SEQ ID NO: 39230 - protein, 9 aa, synthetic construct
GGTGVDVLL

SEQ ID NO: 39231 - protein, 9 aa, synthetic construct
GGTGVDVLN

SEQ ID NO: 39232 - protein, 9 aa, synthetic construct
GGTGVDVLS

SEQ ID NO: 39233 - protein, 9 aa, synthetic construct
GGTGVDVLY

SEQ ID NO: 39234 - protein, 9 aa, synthetic construct
GGTGVDVMA

SEQ ID NO: 39235 - protein, 9 aa, synthetic construct
GGTGVDVMN

SEQ ID NO: 39236 - protein, 9 aa, synthetic construct
GGTGYDRMY

SEQ ID NO: 39237 - protein, 9 aa, synthetic construct
GGTGYDSLA

SEQ ID NO: 39238 - protein, 9 aa, synthetic construct
GGTGYDSLD

SEQ ID NO: 39239 - protein, 9 aa, synthetic construct
GGVGADHLW

SEQ ID NO: 39240 - protein, 9 aa, synthetic construct
GGVGADELY

SEQ ID NO: 39241 - protein, 9 aa, synthetic construct
GGVGADEMS

SEQ ID NO: 39242 - protein, 9 aa, synthetic construct
GGVGADFFV

SEQ ID NO: 39243 - protein, 9 aa, synthetic construct
GGVGADFLA

SEQ ID NO: 39244 - protein, 9 aa, synthetic construct
GGVGADFLH

SEQ ID NO: 39245 - protein, 9 aa, synthetic construct
GGVGADFLK

SEQ ID NO: 39246 - protein, 9 aa, synthetic construct
GGVGADFLS

SEQ ID NO: 39247 - protein, 9 aa, synthetic construct
GGVGADFMA

SEQ ID NO: 39248 - protein, 9 aa, synthetic construct
GGVGADGLA

SEQ ID NO: 39249 - protein, 9 aa, synthetic construct
GGVGADHFV

SEQ ID NO: 39250 - protein, 9 aa, synthetic construct
GGVGADHLI

SEQ ID NO: 39251 - protein, 9 aa, synthetic construct
GGVGADHLN

SEQ ID NO: 39252 - protein, 9 aa, synthetic construct
GGVGADHLV

SEQ ID NO: 39253 - protein, 9 aa, synthetic construct
GGVGADHVF

SEQ ID NO: 39254 - protein, 9 aa, synthetic construct
GGVGADELK

SEQ ID NO: 39255 - protein, 9 aa, synthetic construct
GGVGADIFR

SEQ ID NO: 39256 - protein, 9 aa, synthetic construct
GGVGADIIF

SEQ ID NO: 39257 - protein, 9 aa, synthetic construct
GGVGADIIS

SEQ ID NO: 39258 - protein, 9 aa, synthetic construct
GGVGADIIT

SEQ ID NO: 39259 - protein, 9 aa, synthetic construct
GGVGADILA

SEQ ID NO: 39260 - protein, 9 aa, synthetic construct
GGVGADILQ

SEQ ID NO: 39261 - protein, 9 aa, synthetic construct
GGVGADILV

SEQ ID NO: 39262 - protein, 9 aa, synthetic construct
GGVGADKFV

SEQ ID NO: 39263 - protein, 9 aa, synthetic construct
GGVGADKIT

SEQ ID NO: 39264 - protein, 9 aa, synthetic construct
GGVGADKLM

SEQ ID NO: 39265 - protein, 9 aa, synthetic construct
GGVGADKLW

SEQ ID NO: 39266 - protein, 9 aa, synthetic construct
GGVGADKMD

SEQ ID NO: 39267 - protein, 9 aa, synthetic construct
GGVGADKMS

SEQ ID NO: 39268 - protein, 9 aa, synthetic construct
GGVGADELR

SEQ ID NO: 39269 - protein, 9 aa, synthetic construct
GGVGADELI

SEQ ID NO: 39270 - protein, 9 aa, synthetic construct
GGTGYDSMY

SEQ ID NO: 39271 - protein, 9 aa, synthetic construct
GGTGYDVLL

SEQ ID NO: 39272 - protein, 9 aa, synthetic construct
GGTGYDSVQ

SEQ ID NO: 39273 - protein, 9 aa, synthetic construct
GGTGYDTAV

SEQ ID NO: 39274 - protein, 9 aa, synthetic construct
GGTGYDTFN

SEQ ID NO: 39275 - protein, 9 aa, synthetic construct
GGTGYDTIW

SEQ ID NO: 39276 - protein, 9 aa, synthetic construct
GGTGYDTLA

SEQ ID NO: 39277 - protein, 9 aa, synthetic construct
GGTGYDTLN

SEQ ID NO: 39278 - protein, 9 aa, synthetic construct
GGTGYDTLT

SEQ ID NO: 39279 - protein, 9 aa, synthetic construct
GGTGYDTLV

SEQ ID NO: 39280 - protein, 9 aa, synthetic construct
GGTGYDTME

SEQ ID NO: 39281 - protein, 9 aa, synthetic construct
GGTGYDTML

SEQ ID NO: 39282 - protein, 9 aa, synthetic construct
GGTGYDTVI

SEQ ID NO: 39283 - protein, 9 aa, synthetic construct
GGTGYDVID

SEQ ID NO: 39284 - protein, 9 aa, synthetic construct
GGTGYDVLD

SEQ ID NO: 39285 - protein, 9 aa, synthetic construct
GGTGYDVMD

SEQ ID NO: 39286 - protein, 9 aa, synthetic construct
GGVGADELH

SEQ ID NO: 39287 - protein, 9 aa, synthetic construct
GGTGYDYAI

SEQ ID NO: 39288 - protein, 9 aa, synthetic construct
GGTGYDYLA

SEQ ID NO: 39289 - protein, 9 aa, synthetic construct
GGTGYDYLY

SEQ ID NO: 39290 - protein, 9 aa, synthetic construct
GGVGADAFV

SEQ ID NO: 39291 - protein, 9 aa, synthetic construct
GGVGADAID

SEQ ID NO: 39292 - protein, 9 aa, synthetic construct
GGVGADALE

SEQ ID NO: 39293 - protein, 9 aa, synthetic construct
GGVGADALH

SEQ ID NO: 39294 - protein, 9 aa, synthetic construct
GGVGADALL

SEQ ID NO: 39295 - protein, 9 aa, synthetic construct
GGVGADDFV

SEQ ID NO: 39296 - protein, 9 aa, synthetic construct
GGVGADDLG

SEQ ID NO: 39297 - protein, 9 aa, synthetic construct
GGVGADDLV

SEQ ID NO: 39298 - protein, 9 aa, synthetic construct
GGVGADDMY

SEQ ID NO: 39299 - protein, 9 aa, synthetic construct
GGVGADDYY

SEQ ID NO: 39300 - protein, 9 aa, synthetic construct
GGVGQDSLF

SEQ ID NO: 39301 - protein, 9 aa, synthetic construct
GGVGQDSLH

SEQ ID NO: 39302 - protein, 9 aa, synthetic construct
GGVGQDTAL

SEQ ID NO: 39303 - protein, 9 aa, synthetic construct
GGYGEDTLL

SEQ ID NO: 39304 - protein, 9 aa, synthetic construct
GGYGDDTLH

SEQ ID NO: 39305 - protein, 9 aa, synthetic construct
GGYGDDTLK

SEQ ID NO: 39306 - protein, 9 aa, synthetic construct
GGYGDDTLQ

SEQ ID NO: 39307 - protein, 9 aa, synthetic construct
GGYGDDTMF

SEQ ID NO: 39308 - protein, 9 aa, synthetic construct
GGYGDDVAN

SEQ ID NO: 39309 - protein, 9 aa, synthetic construct
GGYGDDVIA

SEQ ID NO: 39310 - protein, 9 aa, synthetic construct
GGYGDDVIN

SEQ ID NO: 39311 - protein, 9 aa, synthetic construct
GGYGDDVLA

SEQ ID NO: 39312 - protein, 9 aa, synthetic construct
GGYGDDVLG

SEQ ID NO: 39313 - protein, 9 aa, synthetic construct
GGYGDDVLQ

SEQ ID NO: 39314 - protein, 9 aa, synthetic construct
GGYGDDVMD

SEQ ID NO: 39315 - protein, 9 aa, synthetic construct
GGYGDDVMT

SEQ ID NO: 39316 - protein, 9 aa, synthetic construct
GGYGDDVVE

SEQ ID NO: 39317 - protein, 9 aa, synthetic construct
GGYGDDWLI

SEQ ID NO: 39318 - protein, 9 aa, synthetic construct
GGYGDDWLT

SEQ ID NO: 39319 - protein, 9 aa, synthetic construct
GGYGDDYII

SEQ ID NO: 39320 - protein, 9 aa, synthetic construct
GGYGDDYLD

SEQ ID NO: 39321 - protein, 9 aa, synthetic construct
GGYGDDYLG

SEQ ID NO: 39322 - protein, 9 aa, synthetic construct
GGYGEDCLI

SEQ ID NO: 39323 - protein, 9 aa, synthetic construct
GGYGEDIII

SEQ ID NO: 39324 - protein, 9 aa, synthetic construct
GGYGEDILD

SEQ ID NO: 39325 - protein, 9 aa, synthetic construct
GGYGEDILI

SEQ ID NO: 39326 - protein, 9 aa, synthetic construct
GGYGEDILL

SEQ ID NO: 39327 - protein, 9 aa, synthetic construct
GGYGEDLLA

SEQ ID NO: 39328 - protein, 9 aa, synthetic construct
GGYGEDLLT

SEQ ID NO: 39329 - protein, 9 aa, synthetic construct
GGYGEDLVY

SEQ ID NO: 39330 - protein, 9 aa, synthetic construct
GGYGEDQLE

SEQ ID NO: 39331 - protein, 9 aa, synthetic construct
GGYGEDRME

SEQ ID NO: 39332 - protein, 9 aa, synthetic construct
GGYGEDRMF

SEQ ID NO: 39333 - protein, 9 aa, synthetic construct
GGYGDDTIT

SEQ ID NO: 39334 - protein, 9 aa, synthetic construct
GGYGDDTIS

SEQ ID NO: 39335 - protein, 9 aa, synthetic construct
GGYGDDTIL

SEQ ID NO: 39336 - protein, 9 aa, synthetic construct
GGYGDDRLH

SEQ ID NO: 39337 - protein, 9 aa, synthetic construct
GGYGDDNMT

SEQ ID NO: 39338 - protein, 9 aa, synthetic construct
GGYGDDQII

SEQ ID NO: 39339 - protein, 9 aa, synthetic construct
GGYGDDQLD

SEQ ID NO: 39340 - protein, 9 aa, synthetic construct
GGYGDDQLH

SEQ ID NO: 39341 - protein, 9 aa, synthetic construct
GGYGDDQLM

SEQ ID NO: 39342 - protein, 9 aa, synthetic construct
GGYGDDQMH

SEQ ID NO: 39343 - protein, 9 aa, synthetic construct
GGYGDDQYF

SEQ ID NO: 39344 - protein, 9 aa, synthetic construct
GGYGDDRIG

SEQ ID NO: 39345 - protein, 9 aa, synthetic construct
GGYGDDRIV

SEQ ID NO: 39346 - protein, 9 aa, synthetic construct
GGYGDDRIY

SEQ ID NO: 39347 - protein, 9 aa, synthetic construct
GGYGDDRLA

SEQ ID NO: 39348 - protein, 9 aa, synthetic construct
GGYGDDRLF

SEQ ID NO: 39349 - protein, 9 aa, synthetic construct
GGYGDDRLG

SEQ ID NO: 39350 - protein, 9 aa, synthetic construct
GGYGDDRLK

SEQ ID NO: 39351 - protein, 9 aa, synthetic construct
GGYGDDTIH

SEQ ID NO: 39352 - protein, 9 aa, synthetic construct
GGYGDDRLT

SEQ ID NO: 39353 - protein, 9 aa, synthetic construct
GGYGDDRLV

SEQ ID NO: 39354 - protein, 9 aa, synthetic construct
GGYGDDRLY

SEQ ID NO: 39355 - protein, 9 aa, synthetic construct
GGYGDDSIE

SEQ ID NO: 39356 - protein, 9 aa, synthetic construct
GGYGDDSLE

SEQ ID NO: 39357 - protein, 9 aa, synthetic construct
GGYGDDSLM

SEQ ID NO: 39358 - protein, 9 aa, synthetic construct
GGYGDDSLS

SEQ ID NO: 39359 - protein, 9 aa, synthetic construct
GGYGDDSLT

SEQ ID NO: 39360 - protein, 9 aa, synthetic construct
GGYGDDSLV

SEQ ID NO: 39361 - protein, 9 aa, synthetic construct
GGYGDDSLY

SEQ ID NO: 39362 - protein, 9 aa, synthetic construct
GGYGDDTFR

SEQ ID NO: 39363 - protein, 9 aa, synthetic construct
GGYGDDTFY

SEQ ID NO: 39364 - protein, 9 aa, synthetic construct
GGYGDDTIA

SEQ ID NO: 39365 - protein, 9 aa, synthetic construct
GGYGEDTLI

SEQ ID NO: 39366 - protein, 9 aa, synthetic construct
GGYGEDTLS

SEQ ID NO: 39367 - protein, 9 aa, synthetic construct
GGYGLDIAD

SEQ ID NO: 39368 - protein, 9 aa, synthetic construct
GGYGEDYIS

SEQ ID NO: 39369 - protein, 9 aa, synthetic construct
GGYGHDVIE

SEQ ID NO: 39370 - protein, 9 aa, synthetic construct
GGYGIDFMY

SEQ ID NO: 39371 - protein, 9 aa, synthetic construct
GGYGIDHIF

SEQ ID NO: 39372 - protein, 9 aa, synthetic construct
GGYGIDHIH

SEQ ID NO: 39373 - protein, 9 aa, synthetic construct
GGYGIDILQ

SEQ ID NO: 39374 - protein, 9 aa, synthetic construct
GGYGIDKLY

SEQ ID NO: 39375 - protein, 9 aa, synthetic construct
GGYGIDLLN

SEQ ID NO: 39376 - protein, 9 aa, synthetic construct
GGYGIDQLD

SEQ ID NO: 39377 - protein, 9 aa, synthetic construct
GGYGIDQMI

SEQ ID NO: 39378 - protein, 9 aa, synthetic construct
GGYGIDRLY

SEQ ID NO: 39379 - protein, 9 aa, synthetic construct
GGYGIDSLF

SEQ ID NO: 39380 - protein, 9 aa, synthetic construct
GGYGIDSMD

SEQ ID NO: 39381 - protein, 9 aa, synthetic construct
GGYGIDSMS

SEQ ID NO: 39382 - protein, 9 aa, synthetic construct
GGYGIDTLI

SEQ ID NO: 39383 - protein, 9 aa, synthetic construct
GGYGIDTLT

SEQ ID NO: 39384 - protein, 9 aa, synthetic construct
GGYGIDTMD

SEQ ID NO: 39385 - protein, 9 aa, synthetic construct
GGYGIDTVT

SEQ ID NO: 39386 - protein, 9 aa, synthetic construct
GGYGIDWLS

SEQ ID NO: 39387 - protein, 9 aa, synthetic construct
GGYGIDYLT

SEQ ID NO: 39388 - protein, 9 aa, synthetic construct
GGYGKDIIK

SEQ ID NO: 39389 - protein, 9 aa, synthetic construct
GGYGKDILV

SEQ ID NO: 39390 - protein, 9 aa, synthetic construct
GGYGKDLIA

SEQ ID NO: 39391 - protein, 9 aa, synthetic construct
GGYGKDRLE

SEQ ID NO: 39392 - protein, 9 aa, synthetic construct
GGYGKDRLY

SEQ ID NO: 39393 - protein, 9 aa, synthetic construct
GGYGKDSLI

SEQ ID NO: 39394 - protein, 9 aa, synthetic construct
GGYGKDTLD

SEQ ID NO: 39395 - protein, 9 aa, synthetic construct
GGYGKDVFE

SEQ ID NO: 39396 - protein, 9 aa, synthetic construct
GGYGKDVLS

SEQ ID NO: 39397 - protein, 9 aa, synthetic construct
GGYGKDVLV

SEQ ID NO: 39398 - protein, 9 aa, synthetic construct
GGYGHDTLT

SEQ ID NO: 39399 - protein, 9 aa, synthetic construct
GGYGHDTID

SEQ ID NO: 39400 - protein, 9 aa, synthetic construct
GGYGHDSLT

SEQ ID NO: 39401 - protein, 9 aa, synthetic construct
GGYGGDLLH

SEQ ID NO: 39402 - protein, 9 aa, synthetic construct
GGYGFDEAM

SEQ ID NO: 39403 - protein, 9 aa, synthetic construct
GGYGFDFLL

SEQ ID NO: 39404 - protein, 9 aa, synthetic construct
GGYGFDIAL

SEQ ID NO: 39405 - protein, 9 aa, synthetic construct
GGYGFDILF

SEQ ID NO: 39406 - protein, 9 aa, synthetic construct
GGYGFDRLS

SEQ ID NO: 39407 - protein, 9 aa, synthetic construct
GGYGFDTIE

SEQ ID NO: 39408 - protein, 9 aa, synthetic construct
GGYGFDTIW

SEQ ID NO: 39409 - protein, 9 aa, synthetic construct
GGYGFDTLY

SEQ ID NO: 39410 - protein, 9 aa, synthetic construct
GGYGGDDIL

SEQ ID NO: 39411 - protein, 9 aa, synthetic construct
GGYGGDEIL

SEQ ID NO: 39412 - protein, 9 aa, synthetic construct
GGYGGDHLD

SEQ ID NO: 39413 - protein, 9 aa, synthetic construct
GGYGGDIAD

SEQ ID NO: 39414 - protein, 9 aa, synthetic construct
GGYGGDILM

SEQ ID NO: 39415 - protein, 9 aa, synthetic construct
GGYGGDPYG

SEQ ID NO: 39416 - protein, 9 aa, synthetic construct
GGYGHDRLY

SEQ ID NO: 39417 - protein, 9 aa, synthetic construct
GGYGGDQLS

SEQ ID NO: 39418 - protein, 9 aa, synthetic construct
GGYGGDTIN

SEQ ID NO: 39419 - protein, 9 aa, synthetic construct
GGYGGDTLE

SEQ ID NO: 39420 - protein, 9 aa, synthetic construct
GGYGGDTLK

SEQ ID NO: 39421 - protein, 9 aa, synthetic construct
GGYGGDTLV

SEQ ID NO: 39422 - protein, 9 aa, synthetic construct
GGYGGDWLH

SEQ ID NO: 39423 - protein, 9 aa, synthetic construct
GGYGGDYIR

SEQ ID NO: 39424 - protein, 9 aa, synthetic construct
GGYGGDYLQ

SEQ ID NO: 39425 - protein, 9 aa, synthetic construct
GGYGHDLFL

SEQ ID NO: 39426 - protein, 9 aa, synthetic construct
GGYGHDLLY

SEQ ID NO: 39427 - protein, 9 aa, synthetic construct
GGYGHDRIN

SEQ ID NO: 39428 - protein, 9 aa, synthetic construct
GGYGHDRLI

SEQ ID NO: 39429 - protein, 9 aa, synthetic construct
GGYGHDRLN

SEQ ID NO: 39430 - protein, 9 aa, synthetic construct
GGYGDDNLQ

SEQ ID NO: 39431 - protein, 9 aa, synthetic construct
GGYGDDMVD

SEQ ID NO: 39432 - protein, 9 aa, synthetic construct
GGYGDDMLS

SEQ ID NO: 39433 - protein, 9 aa, synthetic construct
GGYGDDMIA

SEQ ID NO: 39434 - protein, 9 aa, synthetic construct
GGYGADHLD

SEQ ID NO: 39435 - protein, 9 aa, synthetic construct
GGYGADIIQ

SEQ ID NO: 39436 - protein, 9 aa, synthetic construct
GGYGADIIY

SEQ ID NO: 39437 - protein, 9 aa, synthetic construct
GGYGADILA

SEQ ID NO: 39438 - protein, 9 aa, synthetic construct
GGYGADILQ

SEQ ID NO: 39439 - protein, 9 aa, synthetic construct
GGYGADILT

SEQ ID NO: 39440 - protein, 9 aa, synthetic construct
GGYGADILW

SEQ ID NO: 39441 - protein, 9 aa, synthetic construct
GGYGADKFQ

SEQ ID NO: 39442 - protein, 9 aa, synthetic construct
GGYGADKLD

SEQ ID NO: 39443 - protein, 9 aa, synthetic construct
GGYGADKLW

SEQ ID NO: 39444 - protein, 9 aa, synthetic construct
GGYGADKMF

SEQ ID NO: 39445 - protein, 9 aa, synthetic construct
GGYGADLIE

SEQ ID NO: 39446 - protein, 9 aa, synthetic construct
GGYGADLLN

SEQ ID NO: 39447 - protein, 9 aa, synthetic construct
GGYGADLLQ

SEQ ID NO: 39448 - protein, 9 aa, synthetic construct
GGYGADLLT

SEQ ID NO: 39449 - protein, 9 aa, synthetic construct
GGYGADMFV

SEQ ID NO: 39450 - protein, 9 aa, synthetic construct
GGYGADMLT

SEQ ID NO: 39451 - protein, 9 aa, synthetic construct
GGYGADNLF

SEQ ID NO: 39452 - protein, 9 aa, synthetic construct
GGYGADNLT

SEQ ID NO: 39453 - protein, 9 aa, synthetic construct
GGYGADQFV

SEQ ID NO: 39454 - protein, 9 aa, synthetic construct
GGYGADQLQ

SEQ ID NO: 39455 - protein, 9 aa, synthetic construct
GGYGADQLS

SEQ ID NO: 39456 - protein, 9 aa, synthetic construct
GGYGADRIA

SEQ ID NO: 39457 - protein, 9 aa, synthetic construct
GGYGADRID

SEQ ID NO: 39458 - protein, 9 aa, synthetic construct
GGYGADRLI

SEQ ID NO: 39459 - protein, 9 aa, synthetic construct
GGYGADRLW

SEQ ID NO: 39460 - protein, 9 aa, synthetic construct
GGYGADSIS

SEQ ID NO: 39461 - protein, 9 aa, synthetic construct
GGYGADSLQ

SEQ ID NO: 39462 - protein, 9 aa, synthetic construct
GGYGADSLS

SEQ ID NO: 39463 - protein, 9 aa, synthetic construct
GGYGADFIQ

SEQ ID NO: 39464 - protein, 9 aa, synthetic construct
GGYGADEMW

SEQ ID NO: 39465 - protein, 9 aa, synthetic construct
GGYGADELN

SEQ ID NO: 39466 - protein, 9 aa, synthetic construct
GGXGDDVIX

SEQ ID NO: 39467 - protein, 9 aa, synthetic construct
GGWGVDTIH

SEQ ID NO: 39468 - protein, 9 aa, synthetic construct
GGWGVDTIN

SEQ ID NO: 39469 - protein, 9 aa, synthetic construct
GGWGVDTIY

SEQ ID NO: 39470 - protein, 9 aa, synthetic construct
GGWGVDTMT

SEQ ID NO: 39471 - protein, 9 aa, synthetic construct
GGWGWDTLD

SEQ ID NO: 39472 - protein, 9 aa, synthetic construct
GGWGWDTMT

SEQ ID NO: 39473 - protein, 9 aa, synthetic construct
GGWGYDEVH

SEQ ID NO: 39474 - protein, 9 aa, synthetic construct
GGWGYDLVN

SEQ ID NO: 39475 - protein, 9 aa, synthetic construct
GGWGYDQLW

SEQ ID NO: 39476 - protein, 9 aa, synthetic construct
GGWGYDRLE

SEQ ID NO: 39477 - protein, 9 aa, synthetic construct
GGWGYDVAF

SEQ ID NO: 39478 - protein, 9 aa, synthetic construct
GGXGDDALS

SEQ ID NO: 39479 - protein, 9 aa, synthetic construct
GGXGDDTLS

SEQ ID NO: 39480 - protein, 9 aa, synthetic construct
GGXGNDKLN

SEQ ID NO: 39481 - protein, 9 aa, synthetic construct
GGYGADEIY

SEQ ID NO: 39482 - protein, 9 aa, synthetic construct
GGXGNDMLL

SEQ ID NO: 39483 - protein, 9 aa, synthetic construct
GGXGNDSFY

SEQ ID NO: 39484 - protein, 9 aa, synthetic construct
GGXGNDSLD

SEQ ID NO: 39485 - protein, 9 aa, synthetic construct
GGXGNDVLS

SEQ ID NO: 39486 - protein, 9 aa, synthetic construct
GGXGRDILD

SEQ ID NO: 39487 - protein, 9 aa, synthetic construct
GGXGSDTMD

SEQ ID NO: 39488 - protein, 9 aa, synthetic construct
GGXGSDXLR

SEQ ID NO: 39489 - protein, 9 aa, synthetic construct
GGXGXDLLL

SEQ ID NO: 39490 - protein, 9 aa, synthetic construct
GGXGXDQLT

SEQ ID NO: 39491 - protein, 9 aa, synthetic construct
GGXGXDSID

SEQ ID NO: 39492 - protein, 9 aa, synthetic construct
GGXGXDTIL

SEQ ID NO: 39493 - protein, 9 aa, synthetic construct
GGYGADAIA

SEQ ID NO: 39494 - protein, 9 aa, synthetic construct
GGYGADALN

SEQ ID NO: 39495 - protein, 9 aa, synthetic construct
GGYGADSVL

SEQ ID NO: 39496 - protein, 9 aa, synthetic construct
GGYGADTFI

SEQ ID NO: 39497 - protein, 9 aa, synthetic construct
GGYGADTID

SEQ ID NO: 39498 - protein, 9 aa, synthetic construct
GGYGDDILI

SEQ ID NO: 39499 - protein, 9 aa, synthetic construct
GGYGDDFIG

SEQ ID NO: 39500 - protein, 9 aa, synthetic construct
GGYGDDFIQ

SEQ ID NO: 39501 - protein, 9 aa, synthetic construct
GGYGDDFIY

SEQ ID NO: 39502 - protein, 9 aa, synthetic construct
GGYGDDFLA

SEQ ID NO: 39503 - protein, 9 aa, synthetic construct
GGYGDDFLD

SEQ ID NO: 39504 - protein, 9 aa, synthetic construct
GGYGDDFLE

SEQ ID NO: 39505 - protein, 9 aa, synthetic construct
GGYGDDHIK

SEQ ID NO: 39506 - protein, 9 aa, synthetic construct
GGYGDDHLI

SEQ ID NO: 39507 - protein, 9 aa, synthetic construct
GGYGDDHLT

SEQ ID NO: 39508 - protein, 9 aa, synthetic construct
GGYGDDHVI

SEQ ID NO: 39509 - protein, 9 aa, synthetic construct
GGYGDDIFI

SEQ ID NO: 39510 - protein, 9 aa, synthetic construct
GGYGDDIIN

SEQ ID NO: 39511 - protein, 9 aa, synthetic construct
GGYGDDIIY

SEQ ID NO: 39512 - protein, 9 aa, synthetic construct
GGYGDDIYE

SEQ ID NO: 39513 - protein, 9 aa, synthetic construct
GGYGDDELF

SEQ ID NO: 39514 - protein, 9 aa, synthetic construct
GGYGDDKLD

SEQ ID NO: 39515 - protein, 9 aa, synthetic construct
GGYGDDKLE

SEQ ID NO: 39516 - protein, 9 aa, synthetic construct
GGYGDDKLI

SEQ ID NO: 39517 - protein, 9 aa, synthetic construct
GGYGDDLFY

SEQ ID NO: 39518 - protein, 9 aa, synthetic construct
GGYGDDLID

SEQ ID NO: 39519 - protein, 9 aa, synthetic construct
GGYGDDLII

SEQ ID NO: 39520 - protein, 9 aa, synthetic construct
GGYGDDLIQ

SEQ ID NO: 39521 - protein, 9 aa, synthetic construct
GGYGDDLLM

SEQ ID NO: 39522 - protein, 9 aa, synthetic construct
GGYGDDLLQ

SEQ ID NO: 39523 - protein, 9 aa, synthetic construct
GGYGDDLLY

SEQ ID NO: 39524 - protein, 9 aa, synthetic construct
GGYGDDLVE

SEQ ID NO: 39525 - protein, 9 aa, synthetic construct
GGYGDDLVN

SEQ ID NO: 39526 - protein, 9 aa, synthetic construct
GGYGDDLVQ

SEQ ID NO: 39527 - protein, 9 aa, synthetic construct
GGYGDDELV

SEQ ID NO: 39528 - protein, 9 aa, synthetic construct
GGYGDDELE

SEQ ID NO: 39529 - protein, 9 aa, synthetic construct
GGYGADTIN

SEQ ID NO: 39530 - protein, 9 aa, synthetic construct
GGYGADVLQ

SEQ ID NO: 39531 - protein, 9 aa, synthetic construct
GGYGADTIQ

SEQ ID NO: 39532 - protein, 9 aa, synthetic construct
GGYGADTIS

SEQ ID NO: 39533 - protein, 9 aa, synthetic construct
GGYGADTLA

SEQ ID NO: 39534 - protein, 9 aa, synthetic construct
GGYGADTLK

SEQ ID NO: 39535 - protein, 9 aa, synthetic construct
GGYGADTLM

SEQ ID NO: 39536 - protein, 9 aa, synthetic construct
GGYGADTLR

SEQ ID NO: 39537 - protein, 9 aa, synthetic construct
GGYGADTMA

SEQ ID NO: 39538 - protein, 9 aa, synthetic construct
GGYGADTME

SEQ ID NO: 39539 - protein, 9 aa, synthetic construct
GGYGADTMN

SEQ ID NO: 39540 - protein, 9 aa, synthetic construct
GGYGADTVQ

SEQ ID NO: 39541 - protein, 9 aa, synthetic construct
GGYGADTYL

SEQ ID NO: 39542 - protein, 9 aa, synthetic construct
GGYGADVIA

SEQ ID NO: 39543 - protein, 9 aa, synthetic construct
GGYGADVLL

SEQ ID NO: 39544 - protein, 9 aa, synthetic construct
GGYGADVLV

SEQ ID NO: 39545 - protein, 9 aa, synthetic construct
GGYGDDELD

SEQ ID NO: 39546 - protein, 9 aa, synthetic construct
GGYGADVMA

SEQ ID NO: 39547 - protein, 9 aa, synthetic construct
GGYGADVMS

SEQ ID NO: 39548 - protein, 9 aa, synthetic construct
GGYGADVMT

SEQ ID NO: 39549 - protein, 9 aa, synthetic construct
GGYGADWLG

SEQ ID NO: 39550 - protein, 9 aa, synthetic construct
GGYGADYFV

SEQ ID NO: 39551 - protein, 9 aa, synthetic construct
GGYGADYLT

SEQ ID NO: 39552 - protein, 9 aa, synthetic construct
GGYGADYVY

SEQ ID NO: 39553 - protein, 9 aa, synthetic construct
GGYGDDAIY

SEQ ID NO: 39554 - protein, 9 aa, synthetic construct
GGYGDDDFH

SEQ ID NO: 39555 - protein, 9 aa, synthetic construct
GGYGDDDLE

SEQ ID NO: 39556 - protein, 9 aa, synthetic construct
GGYGDDDLV

SEQ ID NO: 39557 - protein, 9 aa, synthetic construct
GGYGDDEIF

SEQ ID NO: 39558 - protein, 9 aa, synthetic construct
GGYGDDELA

SEQ ID NO: 39559 - protein, 9 aa, synthetic construct
GGYGKDVVL

SEQ ID NO: 39560 - protein, 9 aa, synthetic construct
GGYGLDIMV

SEQ ID NO: 39561 - protein, 9 aa, synthetic construct
GGVGQDTAV

SEQ ID NO: 39562 - protein, 9 aa, synthetic construct
GGYGSDSIS

SEQ ID NO: 39563 - protein, 9 aa, synthetic construct
GGYGRDTLD

SEQ ID NO: 39564 - protein, 9 aa, synthetic construct
GGYGRDTLK

SEQ ID NO: 39565 - protein, 9 aa, synthetic construct
GGYGRDTLN

SEQ ID NO: 39566 - protein, 9 aa, synthetic construct
GGYGRDTLR

SEQ ID NO: 39567 - protein, 9 aa, synthetic construct
GGYGRDTMT

SEQ ID NO: 39568 - protein, 9 aa, synthetic construct
GGYGRDTVL

SEQ ID NO: 39569 - protein, 9 aa, synthetic construct
GGYGRDVFV

SEQ ID NO: 39570 - protein, 9 aa, synthetic construct
GGYGRDVLE

SEQ ID NO: 39571 - protein, 9 aa, synthetic construct
GGYGRDVLI

SEQ ID NO: 39572 - protein, 9 aa, synthetic construct
GGYGRDYIK

SEQ ID NO: 39573 - protein, 9 aa, synthetic construct
GGYGRDYVE

SEQ ID NO: 39574 - protein, 9 aa, synthetic construct
GGYGSDAIS

SEQ ID NO: 39575 - protein, 9 aa, synthetic construct
GGYGSDDLR

SEQ ID NO: 39576 - protein, 9 aa, synthetic construct
GGYGSDGLH

SEQ ID NO: 39577 - protein, 9 aa, synthetic construct
GGYGSDIFS

SEQ ID NO: 39578 - protein, 9 aa, synthetic construct
GGYGSDILE

SEQ ID NO: 39579 - protein, 9 aa, synthetic construct
GGYGSDKLL

SEQ ID NO: 39580 - protein, 9 aa, synthetic construct
GGYGSDLLS

SEQ ID NO: 39581 - protein, 9 aa, synthetic construct
GGYGSDLLT

SEQ ID NO: 39582 - protein, 9 aa, synthetic construct
GGYGSDLVI

SEQ ID NO: 39583 - protein, 9 aa, synthetic construct
GGYGSDMLI

SEQ ID NO: 39584 - protein, 9 aa, synthetic construct
GGYGSDMMY

SEQ ID NO: 39585 - protein, 9 aa, synthetic construct
GGYGSDNLF

SEQ ID NO: 39586 - protein, 9 aa, synthetic construct
GGYGSDQLF

SEQ ID NO: 39587 - protein, 9 aa, synthetic construct
GGYGSDRFV

SEQ ID NO: 39588 - protein, 9 aa, synthetic construct
GGYGSDRFY

SEQ ID NO: 39589 - protein, 9 aa, synthetic construct
GGYGSDRIH

SEQ ID NO: 39590 - protein, 9 aa, synthetic construct
GGYGSDRLT

SEQ ID NO: 39591 - protein, 9 aa, synthetic construct
GGYGSDRLY

SEQ ID NO: 39592 - protein, 9 aa, synthetic construct
GGYGRDTIE

SEQ ID NO: 39593 - protein, 9 aa, synthetic construct
GGYGRDTID

SEQ ID NO: 39594 - protein, 9 aa, synthetic construct
GGYGRDTFI

SEQ ID NO: 39595 - protein, 9 aa, synthetic construct
GGYGRDHLI

SEQ ID NO: 39596 - protein, 9 aa, synthetic construct
GGYGQDRLF

SEQ ID NO: 39597 - protein, 9 aa, synthetic construct
GGYGQDRLQ

SEQ ID NO: 39598 - protein, 9 aa, synthetic construct
GGYGQDSLD

SEQ ID NO: 39599 - protein, 9 aa, synthetic construct
GGYGQDTLD

SEQ ID NO: 39600 - protein, 9 aa, synthetic construct
GGYGQDTLE

SEQ ID NO: 39601 - protein, 9 aa, synthetic construct
GGYGQDTLY

SEQ ID NO: 39602 - protein, 9 aa, synthetic construct
GGYGQDYLN

SEQ ID NO: 39603 - protein, 9 aa, synthetic construct
GGYGRDALS

SEQ ID NO: 39604 - protein, 9 aa, synthetic construct
GGYGRDAMS

SEQ ID NO: 39605 - protein, 9 aa, synthetic construct
GGYGRDELY

SEQ ID NO: 39606 - protein, 9 aa, synthetic construct
GGYGRDFLD

SEQ ID NO: 39607 - protein, 9 aa, synthetic construct
GGYGRDFLY

SEQ ID NO: 39608 - protein, 9 aa, synthetic construct
GGYGRDGLV

SEQ ID NO: 39609 - protein, 9 aa, synthetic construct
GGYGRDIIY

SEQ ID NO: 39610 - protein, 9 aa, synthetic construct
GGYGRDTAS

SEQ ID NO: 39611 - protein, 9 aa, synthetic construct
GGYGRDILS

SEQ ID NO: 39612 - protein, 9 aa, synthetic construct
GGYGRDILT

SEQ ID NO: 39613 - protein, 9 aa, synthetic construct
GGYGRDLID

SEQ ID NO: 39614 - protein, 9 aa, synthetic construct
GGYGRDLIY

SEQ ID NO: 39615 - protein, 9 aa, synthetic construct
GGYGRDLLK

SEQ ID NO: 39616 - protein, 9 aa, synthetic construct
GGYGRDLMY

SEQ ID NO: 39617 - protein, 9 aa, synthetic construct
GGYGRDLVY

SEQ ID NO: 39618 - protein, 9 aa, synthetic construct
GGYGRDNMS

SEQ ID NO: 39619 - protein, 9 aa, synthetic construct
GGYGRDQIA

SEQ ID NO: 39620 - protein, 9 aa, synthetic construct
GGYGRDQIS

SEQ ID NO: 39621 - protein, 9 aa, synthetic construct
GGYGRDQLS

SEQ ID NO: 39622 - protein, 9 aa, synthetic construct
GGYGRDRVE

SEQ ID NO: 39623 - protein, 9 aa, synthetic construct
GGYGRDSLF

SEQ ID NO: 39624 - protein, 9 aa, synthetic construct
GGYGSDRYL

SEQ ID NO: 39625 - protein, 9 aa, synthetic construct
GGYGSDSLL

SEQ ID NO: 39626 - protein, 9 aa, synthetic construct
GGYGLDQLH

SEQ ID NO: 39627 - protein, 9 aa, synthetic construct
GGYGSDSLV

SEQ ID NO: 39628 - protein, 9 aa, synthetic construct
GGYGTDTLI

SEQ ID NO: 39629 - protein, 9 aa, synthetic construct
GGYGTDTLS

SEQ ID NO: 39630 - protein, 9 aa, synthetic construct
GGYGTDTLT

SEQ ID NO: 39631 - protein, 9 aa, synthetic construct
GGYGTDVLN

SEQ ID NO: 39632 - protein, 9 aa, synthetic construct
GGYGTDWAD

SEQ ID NO: 39633 - protein, 9 aa, synthetic construct
GGYGVDALY

SEQ ID NO: 39634 - protein, 9 aa, synthetic construct
GGYGVDHLH

SEQ ID NO: 39635 - protein, 9 aa, synthetic construct
GGYGVDIIH

SEQ ID NO: 39636 - protein, 9 aa, synthetic construct
GGYGVDILH

SEQ ID NO: 39637 - protein, 9 aa, synthetic construct
GGYGVDLVI

SEQ ID NO: 39638 - protein, 9 aa, synthetic construct
GGYGVDRLH

SEQ ID NO: 39639 - protein, 9 aa, synthetic construct
GGYGVDTIH

SEQ ID NO: 39640 - protein, 9 aa, synthetic construct
GGYGVDTVV

SEQ ID NO: 39641 - protein, 9 aa, synthetic construct
GGYGVDVVS

SEQ ID NO: 39642 - protein, 9 aa, synthetic construct
GGYGVDYIV

SEQ ID NO: 39643 - protein, 9 aa, synthetic construct
GGYGVDYLF

SEQ ID NO: 39644 - protein, 9 aa, synthetic construct
GGYGWDEFA

SEQ ID NO: 39645 - protein, 9 aa, synthetic construct
GGYGWDEFV

SEQ ID NO: 39646 - protein, 9 aa, synthetic construct
GGYGWDKMF

SEQ ID NO: 39647 - protein, 9 aa, synthetic construct
GGYGWDRIF

SEQ ID NO: 39648 - protein, 9 aa, synthetic construct
GGYGWDRLV

SEQ ID NO: 39649 - protein, 9 aa, synthetic construct
GGYGYDELK

SEQ ID NO: 39650 - protein, 9 aa, synthetic construct
GGYGYDFLF

SEQ ID NO: 39651 - protein, 9 aa, synthetic construct
GGYGYDKLV

SEQ ID NO: 39652 - protein, 9 aa, synthetic construct
GGYGYDRIN

SEQ ID NO: 39653 - protein, 9 aa, synthetic construct
GGYGYDRLE

SEQ ID NO: 39654 - protein, 9 aa, synthetic construct
GGYGYDTIH

SEQ ID NO: 39655 - protein, 9 aa, synthetic construct
GGYGYDTLI

SEQ ID NO: 39656 - protein, 9 aa, synthetic construct
GGYGYDTLR

SEQ ID NO: 39657 - protein, 9 aa, synthetic construct
GGYGTDTLD

SEQ ID NO: 39658 - protein, 9 aa, synthetic construct
GGYGTDTIY

SEQ ID NO: 39659 - protein, 9 aa, synthetic construct
GGYGTDTIN

SEQ ID NO: 39660 - protein, 9 aa, synthetic construct
GGYGSDTVY

SEQ ID NO: 39661 - protein, 9 aa, synthetic construct
GGYGSDTII

SEQ ID NO: 39662 - protein, 9 aa, synthetic construct
GGYGSDTIS

SEQ ID NO: 39663 - protein, 9 aa, synthetic construct
GGYGSDTIT

SEQ ID NO: 39664 - protein, 9 aa, synthetic construct
GGYGSDTIY

SEQ ID NO: 39665 - protein, 9 aa, synthetic construct
GGYGSDTLG

SEQ ID NO: 39666 - protein, 9 aa, synthetic construct
GGYGSDTLL

SEQ ID NO: 39667 - protein, 9 aa, synthetic construct
GGYGSDTLM

SEQ ID NO: 39668 - protein, 9 aa, synthetic construct
GGYGSDTLN

SEQ ID NO: 39669 - protein, 9 aa, synthetic construct
GGYGSDTLQ

SEQ ID NO: 39670 - protein, 9 aa, synthetic construct
GGYGSDTLV

SEQ ID NO: 39671 - protein, 9 aa, synthetic construct
GGYGSDTMT

SEQ ID NO: 39672 - protein, 9 aa, synthetic construct
GGYGSDTVE

SEQ ID NO: 39673 - protein, 9 aa, synthetic construct
GGYGSDTVM

SEQ ID NO: 39674 - protein, 9 aa, synthetic construct
GGYGSDVFF

SEQ ID NO: 39675 - protein, 9 aa, synthetic construct
GGYGTDTID

SEQ ID NO: 39676 - protein, 9 aa, synthetic construct
GGYGSDVIF

SEQ ID NO: 39677 - protein, 9 aa, synthetic construct
GGYGSDVIN

SEQ ID NO: 39678 - protein, 9 aa, synthetic construct
GGYGSDVIY

SEQ ID NO: 39679 - protein, 9 aa, synthetic construct
GGYGSDVVR

SEQ ID NO: 39680 - protein, 9 aa, synthetic construct
GGYGSDYID

SEQ ID NO: 39681 - protein, 9 aa, synthetic construct
GGYGSDYLW

SEQ ID NO: 39682 - protein, 9 aa, synthetic construct
GGYGSDYLY

SEQ ID NO: 39683 - protein, 9 aa, synthetic construct
GGYGTDILT

SEQ ID NO: 39684 - protein, 9 aa, synthetic construct
GGYGTDKLL

SEQ ID NO: 39685 - protein, 9 aa, synthetic construct
GGYGTDLLN

SEQ ID NO: 39686 - protein, 9 aa, synthetic construct
GGYGTDQLT

SEQ ID NO: 39687 - protein, 9 aa, synthetic construct
GGYGTDRLE

SEQ ID NO: 39688 - protein, 9 aa, synthetic construct
GGYGTDTAF

SEQ ID NO: 39689 - protein, 9 aa, synthetic construct
GGYGQDRLE

SEQ ID NO: 39690 - protein, 9 aa, synthetic construct
GGYGQDLLT

SEQ ID NO: 39691 - protein, 9 aa, synthetic construct
GGYGQDILR

SEQ ID NO: 39692 - protein, 9 aa, synthetic construct
GGYGQDFMY

SEQ ID NO: 39693 - protein, 9 aa, synthetic construct
GGYGNDIIS

SEQ ID NO: 39694 - protein, 9 aa, synthetic construct
GGYGNDIIY

SEQ ID NO: 39695 - protein, 9 aa, synthetic construct
GGYGNDILA

SEQ ID NO: 39696 - protein, 9 aa, synthetic construct
GGYGNDILE

SEQ ID NO: 39697 - protein, 9 aa, synthetic construct
GGYGNDILF

SEQ ID NO: 39698 - protein, 9 aa, synthetic construct
GGYGNDILK

SEQ ID NO: 39699 - protein, 9 aa, synthetic construct
GGYGNDILL

SEQ ID NO: 39700 - protein, 9 aa, synthetic construct
GGYGNDILW

SEQ ID NO: 39701 - protein, 9 aa, synthetic construct
GGYGNDIVK

SEQ ID NO: 39702 - protein, 9 aa, synthetic construct
GGYGNDIVY

SEQ ID NO: 39703 - protein, 9 aa, synthetic construct
GGYGNDIYD

SEQ ID NO: 39704 - protein, 9 aa, synthetic construct
GGYGNDKIT

SEQ ID NO: 39705 - protein, 9 aa, synthetic construct
GGYGNDKLD

SEQ ID NO: 39706 - protein, 9 aa, synthetic construct
GGYGNDKLE

SEQ ID NO: 39707 - protein, 9 aa, synthetic construct
GGYGNDKLN

SEQ ID NO: 39708 - protein, 9 aa, synthetic construct
GGYGNDKLS

SEQ ID NO: 39709 - protein, 9 aa, synthetic construct
GGYGNDKLW

SEQ ID NO: 39710 - protein, 9 aa, synthetic construct
GGYGNDKVY

SEQ ID NO: 39711 - protein, 9 aa, synthetic construct
GGYGNDLFY

SEQ ID NO: 39712 - protein, 9 aa, synthetic construct
GGYGNDLID

SEQ ID NO: 39713 - protein, 9 aa, synthetic construct
GGYGNDLIV

SEQ ID NO: 39714 - protein, 9 aa, synthetic construct
GGYGNDLLI

SEQ ID NO: 39715 - protein, 9 aa, synthetic construct
GGYGNDLLN

SEQ ID NO: 39716 - protein, 9 aa, synthetic construct
GGYGNDLLR

SEQ ID NO: 39717 - protein, 9 aa, synthetic construct
GGYGNDLLT

SEQ ID NO: 39718 - protein, 9 aa, synthetic construct
GGYGNDLVY

SEQ ID NO: 39719 - protein, 9 aa, synthetic construct
GGYGNDLYL

SEQ ID NO: 39720 - protein, 9 aa, synthetic construct
GGYGNDLYN

SEQ ID NO: 39721 - protein, 9 aa, synthetic construct
GGYGNDLYR

SEQ ID NO: 39722 - protein, 9 aa, synthetic construct
GGYGNDIIA

SEQ ID NO: 39723 - protein, 9 aa, synthetic construct
GGYGNDIFD

SEQ ID NO: 39724 - protein, 9 aa, synthetic construct
GGYGNDHLF

SEQ ID NO: 39725 - protein, 9 aa, synthetic construct
GGYGNDDVS

SEQ ID NO: 39726 - protein, 9 aa, synthetic construct
GGYGLDTLG

SEQ ID NO: 39727 - protein, 9 aa, synthetic construct
GGYGLDTLS

SEQ ID NO: 39728 - protein, 9 aa, synthetic construct
GGYGLDVIY

SEQ ID NO: 39729 - protein, 9 aa, synthetic construct
GGYGMDRLF

SEQ ID NO: 39730 - protein, 9 aa, synthetic construct
GGYGMDSLE

SEQ ID NO: 39731 - protein, 9 aa, synthetic construct
GGYGMDVLY

SEQ ID NO: 39732 - protein, 9 aa, synthetic construct
GGYGNDALL

SEQ ID NO: 39733 - protein, 9 aa, synthetic construct
GGYGNDALS

SEQ ID NO: 39734 - protein, 9 aa, synthetic construct
GGYGNDALT

SEQ ID NO: 39735 - protein, 9 aa, synthetic construct
GGYGNDAMY

SEQ ID NO: 39736 - protein, 9 aa, synthetic construct
GGYGNDDFH

SEQ ID NO: 39737 - protein, 9 aa, synthetic construct
GGYGNDDLR

SEQ ID NO: 39738 - protein, 9 aa, synthetic construct
GGYGNDDMF

SEQ ID NO: 39739 - protein, 9 aa, synthetic construct
GGYGNDEIF

SEQ ID NO: 39740 - protein, 9 aa, synthetic construct
GGYGNDHIT

SEQ ID NO: 39741 - protein, 9 aa, synthetic construct
GGYGNDEIR

SEQ ID NO: 39742 - protein, 9 aa, synthetic construct
GGYGNDELH

SEQ ID NO: 39743 - protein, 9 aa, synthetic construct
GGYGNDELS

SEQ ID NO: 39744 - protein, 9 aa, synthetic construct
GGYGNDEMN

SEQ ID NO: 39745 - protein, 9 aa, synthetic construct
GGYGNDEVN

SEQ ID NO: 39746 - protein, 9 aa, synthetic construct
GGYGNDEVR

SEQ ID NO: 39747 - protein, 9 aa, synthetic construct
GGYGNDFID

SEQ ID NO: 39748 - protein, 9 aa, synthetic construct
GGYGNDFLE

SEQ ID NO: 39749 - protein, 9 aa, synthetic construct
GGYGNDFLF

SEQ ID NO: 39750 - protein, 9 aa, synthetic construct
GGYGNDFLK

SEQ ID NO: 39751 - protein, 9 aa, synthetic construct
GGYGNDFLL

SEQ ID NO: 39752 - protein, 9 aa, synthetic construct
GGYGNDFLN

SEQ ID NO: 39753 - protein, 9 aa, synthetic construct
GGYGNDFMV

SEQ ID NO: 39754 - protein, 9 aa, synthetic construct
GGYGNDMLH

SEQ ID NO: 39755 - protein, 9 aa, synthetic construct
GGYGNDMLI

SEQ ID NO: 39756 - protein, 9 aa, synthetic construct
GGYGNDMLR

SEQ ID NO: 39757 - protein, 9 aa, synthetic construct
GGYGNDVLA

SEQ ID NO: 39758 - protein, 9 aa, synthetic construct
GGYGNDTFV

SEQ ID NO: 39759 - protein, 9 aa, synthetic construct
GGYGNDTIA

SEQ ID NO: 39760 - protein, 9 aa, synthetic construct
GGYGNDTIF

SEQ ID NO: 39761 - protein, 9 aa, synthetic construct
GGYGNDTLA

SEQ ID NO: 39762 - protein, 9 aa, synthetic construct
GGYGNDTLF

SEQ ID NO: 39763 - protein, 9 aa, synthetic construct
GGYGNDTLM

SEQ ID NO: 39764 - protein, 9 aa, synthetic construct
GGYGNDTMI

SEQ ID NO: 39765 - protein, 9 aa, synthetic construct
GGYGNDTML

SEQ ID NO: 39766 - protein, 9 aa, synthetic construct
GGYGNDTVL

SEQ ID NO: 39767 - protein, 9 aa, synthetic construct
GGYGNDTVV

SEQ ID NO: 39768 - protein, 9 aa, synthetic construct
GGYGNDTYW

SEQ ID NO: 39769 - protein, 9 aa, synthetic construct
GGYGNDVIG

SEQ ID NO: 39770 - protein, 9 aa, synthetic construct
GGYGNDVIK

SEQ ID NO: 39771 - protein, 9 aa, synthetic construct
GGYGNDVLF

SEQ ID NO: 39772 - protein, 9 aa, synthetic construct
GGYGNDSYV

SEQ ID NO: 39773 - protein, 9 aa, synthetic construct
GGYGNDVLQ

SEQ ID NO: 39774 - protein, 9 aa, synthetic construct
GGYGNDVLR

SEQ ID NO: 39775 - protein, 9 aa, synthetic construct
GGYGNDVMR

SEQ ID NO: 39776 - protein, 9 aa, synthetic construct
GGYGNDVVV

SEQ ID NO: 39777 - protein, 9 aa, synthetic construct
GGYGNDWLT

SEQ ID NO: 39778 - protein, 9 aa, synthetic construct
GGYGNDWLV

SEQ ID NO: 39779 - protein, 9 aa, synthetic construct
GGYGNDYIR

SEQ ID NO: 39780 - protein, 9 aa, synthetic construct
GGYGNDYLK

SEQ ID NO: 39781 - protein, 9 aa, synthetic construct
GGYGNDYLR

SEQ ID NO: 39782 - protein, 9 aa, synthetic construct
GGYGNDYLS

SEQ ID NO: 39783 - protein, 9 aa, synthetic construct
GGYGNDYMD

SEQ ID NO: 39784 - protein, 9 aa, synthetic construct
GGYGNDYVY

SEQ ID NO: 39785 - protein, 9 aa, synthetic construct
GGYGPDLVY

SEQ ID NO: 39786 - protein, 9 aa, synthetic construct
GGYGNDTFI

SEQ ID NO: 39787 - protein, 9 aa, synthetic construct
GGYGNDSMV

SEQ ID NO: 39788 - protein, 9 aa, synthetic construct
GGYGNDMLT

SEQ ID NO: 39789 - protein, 9 aa, synthetic construct
GGYGNDRFD

SEQ ID NO: 39790 - protein, 9 aa, synthetic construct
GGYGNDMLY

SEQ ID NO: 39791 - protein, 9 aa, synthetic construct
GGYGNDNIF

SEQ ID NO: 39792 - protein, 9 aa, synthetic construct
GGYGNDNIY

SEQ ID NO: 39793 - protein, 9 aa, synthetic construct
GGYGNDNLF

SEQ ID NO: 39794 - protein, 9 aa, synthetic construct
GGYGNDNLK

SEQ ID NO: 39795 - protein, 9 aa, synthetic construct
GGYGNDNLY

SEQ ID NO: 39796 - protein, 9 aa, synthetic construct
GGYGNDNVQ

SEQ ID NO: 39797 - protein, 9 aa, synthetic construct
GGYGNDQIM

SEQ ID NO: 39798 - protein, 9 aa, synthetic construct
GGYGNDQIN

SEQ ID NO: 39799 - protein, 9 aa, synthetic construct
GGYGNDQLF

SEQ ID NO: 39800 - protein, 9 aa, synthetic construct
GGYGNDQLI

SEQ ID NO: 39801 - protein, 9 aa, synthetic construct
GGYGNDQLV

SEQ ID NO: 39802 - protein, 9 aa, synthetic construct
GGYGNDQMT

SEQ ID NO: 39803 - protein, 9 aa, synthetic construct
GGYGNDRII

SEQ ID NO: 39804 - protein, 9 aa, synthetic construct
GGYGNDSMF

SEQ ID NO: 39805 - protein, 9 aa, synthetic construct
GGYGNDRIN

SEQ ID NO: 39806 - protein, 9 aa, synthetic construct
GGYGNDRIV

SEQ ID NO: 39807 - protein, 9 aa, synthetic construct
GGYGNDRLD

SEQ ID NO: 39808 - protein, 9 aa, synthetic construct
GGYGNDRLE

SEQ ID NO: 39809 - protein, 9 aa, synthetic construct
GGYGNDRLF

SEQ ID NO: 39810 - protein, 9 aa, synthetic construct
GGYGNDRLH

SEQ ID NO: 39811 - protein, 9 aa, synthetic construct
GGYGNDRLS

SEQ ID NO: 39812 - protein, 9 aa, synthetic construct
GGYGNDRVT

SEQ ID NO: 39813 - protein, 9 aa, synthetic construct
GGYGNDRYI

SEQ ID NO: 39814 - protein, 9 aa, synthetic construct
GGYGNDSIY

SEQ ID NO: 39815 - protein, 9 aa, synthetic construct
GGYGNDSLH

SEQ ID NO: 39816 - protein, 9 aa, synthetic construct
GGYGNDSLM

SEQ ID NO: 39817 - protein, 9 aa, synthetic construct
GGYGNDSLT

SEQ ID NO: 39818 - protein, 9 aa, synthetic construct
GGWGVDSLE

SEQ ID NO: 39819 - protein, 9 aa, synthetic construct
GGWGVDELY

SEQ ID NO: 39820 - protein, 9 aa, synthetic construct
GGWGVDALT

SEQ ID NO: 39821 - protein, 9 aa, synthetic construct
GGVGVDRIE

SEQ ID NO: 39822 - protein, 9 aa, synthetic construct
GGVGTDTID

SEQ ID NO: 39823 - protein, 9 aa, synthetic construct
GGVGTDTIS

SEQ ID NO: 39824 - protein, 9 aa, synthetic construct
GGVGTDTLK

SEQ ID NO: 39825 - protein, 9 aa, synthetic construct
GGVGTDTLR

SEQ ID NO: 39826 - protein, 9 aa, synthetic construct
GGVGTDTMR

SEQ ID NO: 39827 - protein, 9 aa, synthetic construct
GGVGTDTVF

SEQ ID NO: 39828 - protein, 9 aa, synthetic construct
GGVGTDTVL

SEQ ID NO: 39829 - protein, 9 aa, synthetic construct
GGVGTDTVS

SEQ ID NO: 39830 - protein, 9 aa, synthetic construct
GGVGTDTVV

SEQ ID NO: 39831 - protein, 9 aa, synthetic construct
GGVGTDVAV

SEQ ID NO: 39832 - protein, 9 aa, synthetic construct
GGVGTDYLS

SEQ ID NO: 39833 - protein, 9 aa, synthetic construct
GGVGVDAAD

SEQ ID NO: 39834 - protein, 9 aa, synthetic construct
GGVGVDALT

SEQ ID NO: 39835 - protein, 9 aa, synthetic construct
GGVGVDFLD

SEQ ID NO: 39836 - protein, 9 aa, synthetic construct
GGVGVDGAA

SEQ ID NO: 39837 - protein, 9 aa, synthetic construct
GGVGVDGLF

SEQ ID NO: 39838 - protein, 9 aa, synthetic construct
GGVGVDHLD

SEQ ID NO: 39839 - protein, 9 aa, synthetic construct
GGVGVDILQ

SEQ ID NO: 39840 - protein, 9 aa, synthetic construct
GGVGVDIYK

SEQ ID NO: 39841 - protein, 9 aa, synthetic construct
GGVGVDKLI

SEQ ID NO: 39842 - protein, 9 aa, synthetic construct
GGVGVDLLG

SEQ ID NO: 39843 - protein, 9 aa, synthetic construct
GGVGVDLMQ

SEQ ID NO: 39844 - protein, 9 aa, synthetic construct
GGVGVDMLF

SEQ ID NO: 39845 - protein, 9 aa, synthetic construct
GGVGVDNLG

SEQ ID NO: 39846 - protein, 9 aa, synthetic construct
GGVGVDNLT

SEQ ID NO: 39847 - protein, 9 aa, synthetic construct
GGVGVDQLT

SEQ ID NO: 39848 - protein, 9 aa, synthetic construct
GGVGVDQLY

SEQ ID NO: 39849 - protein, 9 aa, synthetic construct
GGVGVDRAD

SEQ ID NO: 39850 - protein, 9 aa, synthetic construct
GGVGVDRFI

SEQ ID NO: 39851 - protein, 9 aa, synthetic construct
GGVGTDTAF

SEQ ID NO: 39852 - protein, 9 aa, synthetic construct
GGVGTDTAA

SEQ ID NO: 39853 - protein, 9 aa, synthetic construct
GGVGTDSVT

SEQ ID NO: 39854 - protein, 9 aa, synthetic construct
GGVGTDILD

SEQ ID NO: 39855 - protein, 9 aa, synthetic construct
GGVGSDWLF

SEQ ID NO: 39856 - protein, 9 aa, synthetic construct
GGVGSDYFD

SEQ ID NO: 39857 - protein, 9 aa, synthetic construct
GGVGSDYLK

SEQ ID NO: 39858 - protein, 9 aa, synthetic construct
GGVGSDYLM

SEQ ID NO: 39859 - protein, 9 aa, synthetic construct
GGVGSDYLQ

SEQ ID NO: 39860 - protein, 9 aa, synthetic construct
GGVGSDYLT

SEQ ID NO: 39861 - protein, 9 aa, synthetic construct
GGVGSDYVF

SEQ ID NO: 39862 - protein, 9 aa, synthetic construct
GGVGTDALD

SEQ ID NO: 39863 - protein, 9 aa, synthetic construct
GGVGTDALT

SEQ ID NO: 39864 - protein, 9 aa, synthetic construct
GGVGTDDLY

SEQ ID NO: 39865 - protein, 9 aa, synthetic construct
GGVGTDELF

SEQ ID NO: 39866 - protein, 9 aa, synthetic construct
GGVGTDELY

SEQ ID NO: 39867 - protein, 9 aa, synthetic construct
GGVGTDIAV

SEQ ID NO: 39868 - protein, 9 aa, synthetic construct
GGVGTDIMA

SEQ ID NO: 39869 - protein, 9 aa, synthetic construct
GGVGTDSVF

SEQ ID NO: 39870 - protein, 9 aa, synthetic construct
GGVGTDIMN

SEQ ID NO: 39871 - protein, 9 aa, synthetic construct
GGVGTDIVD

SEQ ID NO: 39872 - protein, 9 aa, synthetic construct
GGVGTDKLT

SEQ ID NO: 39873 - protein, 9 aa, synthetic construct
GGVGTDKLY

SEQ ID NO: 39874 - protein, 9 aa, synthetic construct
GGVGTDMLT

SEQ ID NO: 39875 - protein, 9 aa, synthetic construct
GGVGTDNLL

SEQ ID NO: 39876 - protein, 9 aa, synthetic construct
GGVGTDNLT

SEQ ID NO: 39877 - protein, 9 aa, synthetic construct
GGVGTDRIL

SEQ ID NO: 39878 - protein, 9 aa, synthetic construct
GGVGTDRLE

SEQ ID NO: 39879 - protein, 9 aa, synthetic construct
GGVGTDRLF

SEQ ID NO: 39880 - protein, 9 aa, synthetic construct
GGVGTDSLA

SEQ ID NO: 39881 - protein, 9 aa, synthetic construct
GGVGTDSLR

SEQ ID NO: 39882 - protein, 9 aa, synthetic construct
GGVGTDSLV

SEQ ID NO: 39883 - protein, 9 aa, synthetic construct
GGVGVDRFV

SEQ ID NO: 39884 - protein, 9 aa, synthetic construct
GGVGVDRLN

SEQ ID NO: 39885 - protein, 9 aa, synthetic construct
GGWGTDTLL

SEQ ID NO: 39886 - protein, 9 aa, synthetic construct
GGVGVDRML

SEQ ID NO: 39887 - protein, 9 aa, synthetic construct
GGWGADILN

SEQ ID NO: 39888 - protein, 9 aa, synthetic construct
GGWGADILR

SEQ ID NO: 39889 - protein, 9 aa, synthetic construct
GGWGADLLD

SEQ ID NO: 39890 - protein, 9 aa, synthetic construct
GGWGADLLV

SEQ ID NO: 39891 - protein, 9 aa, synthetic construct
GGWGADNLD

SEQ ID NO: 39892 - protein, 9 aa, synthetic construct
GGWGADNLF

SEQ ID NO: 39893 - protein, 9 aa, synthetic construct
GGWGADNLY

SEQ ID NO: 39894 - protein, 9 aa, synthetic construct
GGWGADQLI

SEQ ID NO: 39895 - protein, 9 aa, synthetic construct
GGWGADRFH

SEQ ID NO: 39896 - protein, 9 aa, synthetic construct
GGWGADRFS

SEQ ID NO: 39897 - protein, 9 aa, synthetic construct
GGWGADRLD

SEQ ID NO: 39898 - protein, 9 aa, synthetic construct
GGWGADRLH

SEQ ID NO: 39899 - protein, 9 aa, synthetic construct
GGWGADRLI

SEQ ID NO: 39900 - protein, 9 aa, synthetic construct
GGWGADRLN

SEQ ID NO: 39901 - protein, 9 aa, synthetic construct
GGWGADRME

SEQ ID NO: 39902 - protein, 9 aa, synthetic construct
GGWGADRMS

SEQ ID NO: 39903 - protein, 9 aa, synthetic construct
GGWGADRMV

SEQ ID NO: 39904 - protein, 9 aa, synthetic construct
GGWGADSFV

SEQ ID NO: 39905 - protein, 9 aa, synthetic construct
GGWGADSLA

SEQ ID NO: 39906 - protein, 9 aa, synthetic construct
GGWGADSLS

SEQ ID NO: 39907 - protein, 9 aa, synthetic construct
GGWGADSMD

SEQ ID NO: 39908 - protein, 9 aa, synthetic construct
GGWGADTFV

SEQ ID NO: 39909 - protein, 9 aa, synthetic construct
GGWGADTII

SEQ ID NO: 39910 - protein, 9 aa, synthetic construct
GGWGADTLE

SEQ ID NO: 39911 - protein, 9 aa, synthetic construct
GGWGADTLK

SEQ ID NO: 39912 - protein, 9 aa, synthetic construct
GGWGADTMV

SEQ ID NO: 39913 - protein, 9 aa, synthetic construct
GGWGADTMY

SEQ ID NO: 39914 - protein, 9 aa, synthetic construct
GGWGADVFR

SEQ ID NO: 39915 - protein, 9 aa, synthetic construct
GGWGADVLD

SEQ ID NO: 39916 - protein, 9 aa, synthetic construct
GGWGADHLT

SEQ ID NO: 39917 - protein, 9 aa, synthetic construct
GGWGADHFV

SEQ ID NO: 39918 - protein, 9 aa, synthetic construct
GGWGADELY

SEQ ID NO: 39919 - protein, 9 aa, synthetic construct
GGVGVDVMT

SEQ ID NO: 39920 - protein, 9 aa, synthetic construct
GGVGVDSIN

SEQ ID NO: 39921 - protein, 9 aa, synthetic construct
GGVGVDSLD

SEQ ID NO: 39922 - protein, 9 aa, synthetic construct
GGVGVDSMA

SEQ ID NO: 39923 - protein, 9 aa, synthetic construct
GGVGVDSYD

SEQ ID NO: 39924 - protein, 9 aa, synthetic construct
GGVGVDTIS

SEQ ID NO: 39925 - protein, 9 aa, synthetic construct
GGVGVDTLK

SEQ ID NO: 39926 - protein, 9 aa, synthetic construct
GGVGVDTLL

SEQ ID NO: 39927 - protein, 9 aa, synthetic construct
GGVGVDTLM

SEQ ID NO: 39928 - protein, 9 aa, synthetic construct
GGVGVDTLQ

SEQ ID NO: 39929 - protein, 9 aa, synthetic construct
GGVGVDTLR

SEQ ID NO: 39930 - protein, 9 aa, synthetic construct
GGVGVDTLS

SEQ ID NO: 39931 - protein, 9 aa, synthetic construct
GGVGVDTLY

SEQ ID NO: 39932 - protein, 9 aa, synthetic construct
GGVGVDTMD

SEQ ID NO: 39933 - protein, 9 aa, synthetic construct
GGVGYDDIY

SEQ ID NO: 39934 - protein, 9 aa, synthetic construct
GGWGADELN

SEQ ID NO: 39935 - protein, 9 aa, synthetic construct
GGVGYDELT

SEQ ID NO: 39936 - protein, 9 aa, synthetic construct
GGVGYDILD

SEQ ID NO: 39937 - protein, 9 aa, synthetic construct
GGVGYDILE

SEQ ID NO: 39938 - protein, 9 aa, synthetic construct
GGVGYDILY

SEQ ID NO: 39939 - protein, 9 aa, synthetic construct
GGVGYDKLY

SEQ ID NO: 39940 - protein, 9 aa, synthetic construct
GGVGYDRLY

SEQ ID NO: 39941 - protein, 9 aa, synthetic construct
GGVGYDSLT

SEQ ID NO: 39942 - protein, 9 aa, synthetic construct
GGVGYDTLN

SEQ ID NO: 39943 - protein, 9 aa, synthetic construct
GGVGYDTLY

SEQ ID NO: 39944 - protein, 9 aa, synthetic construct
GGVGYDVLE

SEQ ID NO: 39945 - protein, 9 aa, synthetic construct
GGVGYDVLH

SEQ ID NO: 39946 - protein, 9 aa, synthetic construct
GGVGYDVLI

SEQ ID NO: 39947 - protein, 9 aa, synthetic construct
GGWGADDLI

SEQ ID NO: 39948 - protein, 9 aa, synthetic construct
GGVGSDWAS

SEQ ID NO: 39949 - protein, 9 aa, synthetic construct
GGVGSDVLR

SEQ ID NO: 39950 - protein, 9 aa, synthetic construct
GGVGSDVLA

SEQ ID NO: 39951 - protein, 9 aa, synthetic construct
GGVGSDVII

SEQ ID NO: 39952 - protein, 9 aa, synthetic construct
GGVGRDMLL

SEQ ID NO: 39953 - protein, 9 aa, synthetic construct
GGVGRDNLI

SEQ ID NO: 39954 - protein, 9 aa, synthetic construct
GGVGRDQFH

SEQ ID NO: 39955 - protein, 9 aa, synthetic construct
GGVGRDQIH

SEQ ID NO: 39956 - protein, 9 aa, synthetic construct
GGVGRDQLI

SEQ ID NO: 39957 - protein, 9 aa, synthetic construct
GGVGRDQLY

SEQ ID NO: 39958 - protein, 9 aa, synthetic construct
GGVGRDQMT

SEQ ID NO: 39959 - protein, 9 aa, synthetic construct
GGVGRDRLN

SEQ ID NO: 39960 - protein, 9 aa, synthetic construct
GGVGRDRLS

SEQ ID NO: 39961 - protein, 9 aa, synthetic construct
GGVGRDRVV

SEQ ID NO: 39962 - protein, 9 aa, synthetic construct
GGVGRDSIT

SEQ ID NO: 39963 - protein, 9 aa, synthetic construct
GGVGRDTFI

SEQ ID NO: 39964 - protein, 9 aa, synthetic construct
GGVGRDTFS

SEQ ID NO: 39965 - protein, 9 aa, synthetic construct
GGVGRDTID

SEQ ID NO: 39966 - protein, 9 aa, synthetic construct
GGVGRDTIL

SEQ ID NO: 39967 - protein, 9 aa, synthetic construct
GGVGRDTLK

SEQ ID NO: 39968 - protein, 9 aa, synthetic construct
GGVGRDTLY

SEQ ID NO: 39969 - protein, 9 aa, synthetic construct
GGVGRDTYK

SEQ ID NO: 39970 - protein, 9 aa, synthetic construct
GGVGRDVLA

SEQ ID NO: 39971 - protein, 9 aa, synthetic construct
GGVGRDVLD

SEQ ID NO: 39972 - protein, 9 aa, synthetic construct
GGVGRDVLS

SEQ ID NO: 39973 - protein, 9 aa, synthetic construct
GGVGRDYLA

SEQ ID NO: 39974 - protein, 9 aa, synthetic construct
GGVGRDYLD

SEQ ID NO: 39975 - protein, 9 aa, synthetic construct
GGVGRDYMD

SEQ ID NO: 39976 - protein, 9 aa, synthetic construct
GGVGSDAIY

SEQ ID NO: 39977 - protein, 9 aa, synthetic construct
GGVGSDALW

SEQ ID NO: 39978 - protein, 9 aa, synthetic construct
GGVGSDDIQ

SEQ ID NO: 39979 - protein, 9 aa, synthetic construct
GGVGSDDLR

SEQ ID NO: 39980 - protein, 9 aa, synthetic construct
GGVGSDDLY

SEQ ID NO: 39981 - protein, 9 aa, synthetic construct
GGVGRDLMT

SEQ ID NO: 39982 - protein, 9 aa, synthetic construct
GGVGRDLLI

SEQ ID NO: 39983 - protein, 9 aa, synthetic construct
GGVGRDLLF

SEQ ID NO: 39984 - protein, 9 aa, synthetic construct
GGVGRDALS

SEQ ID NO: 39985 - protein, 9 aa, synthetic construct
GGVGQDTID

SEQ ID NO: 39986 - protein, 9 aa, synthetic construct
GGVGQDTIF

SEQ ID NO: 39987 - protein, 9 aa, synthetic construct
GGVGQDTLR

SEQ ID NO: 39988 - protein, 9 aa, synthetic construct
GGVGQDTLW

SEQ ID NO: 39989 - protein, 9 aa, synthetic construct
GGVGQDTMV

SEQ ID NO: 39990 - protein, 9 aa, synthetic construct
GGVGQDTYH

SEQ ID NO: 39991 - protein, 9 aa, synthetic construct
GGVGQDVLI

SEQ ID NO: 39992 - protein, 9 aa, synthetic construct
GGVGQDVLT

SEQ ID NO: 39993 - protein, 9 aa, synthetic construct
GGVGQDVLY

SEQ ID NO: 39994 - protein, 9 aa, synthetic construct
GGVGQDYLA

SEQ ID NO: 39995 - protein, 9 aa, synthetic construct
GGVGQDYLD

SEQ ID NO: 39996 - protein, 9 aa, synthetic construct
GGVGRDALA

SEQ ID NO: 39997 - protein, 9 aa, synthetic construct
GGVGRDALF

SEQ ID NO: 39998 - protein, 9 aa, synthetic construct
GGVGRDDIR

SEQ ID NO: 39999 - protein, 9 aa, synthetic construct
GGVGRDLLD

SEQ ID NO: 40000 - protein, 9 aa, synthetic construct
GGVGRDDLF

SEQ ID NO: 40001 - protein, 9 aa, synthetic construct
GGVGRDDLY

SEQ ID NO: 40002 - protein, 9 aa, synthetic construct
GGVGRDEIH

SEQ ID NO: 40003 - protein, 9 aa, synthetic construct
GGVGRDEIL

SEQ ID NO: 40004 - protein, 9 aa, synthetic construct
GGVGRDGLA

SEQ ID NO: 40005 - protein, 9 aa, synthetic construct
GGVGRDHLA

SEQ ID NO: 40006 - protein, 9 aa, synthetic construct
GGVGRDIIL

SEQ ID NO: 40007 - protein, 9 aa, synthetic construct
GGVGRDILH

SEQ ID NO: 40008 - protein, 9 aa, synthetic construct
GGVGRDILI

SEQ ID NO: 40009 - protein, 9 aa, synthetic construct
GGVGRDILR

SEQ ID NO: 40010 - protein, 9 aa, synthetic construct
GGVGRDIMT

SEQ ID NO: 40011 - protein, 9 aa, synthetic construct
GGVGRDKLF

SEQ ID NO: 40012 - protein, 9 aa, synthetic construct
GGVGRDKLQ

SEQ ID NO: 40013 - protein, 9 aa, synthetic construct
GGVGSDEIF

SEQ ID NO: 40014 - protein, 9 aa, synthetic construct
GGVGSDEIY

SEQ ID NO: 40015 - protein, 9 aa, synthetic construct
GGVGSDFIT

SEQ ID NO: 40016 - protein, 9 aa, synthetic construct
GGVGSDTAF

SEQ ID NO: 40017 - protein, 9 aa, synthetic construct
GGVGSDRLW

SEQ ID NO: 40018 - protein, 9 aa, synthetic construct
GGVGSDRME

SEQ ID NO: 40019 - protein, 9 aa, synthetic construct
GGVGSDRYV

SEQ ID NO: 40020 - protein, 9 aa, synthetic construct
GGVGSDSFI

SEQ ID NO: 40021 - protein, 9 aa, synthetic construct
GGVGSDSID

SEQ ID NO: 40022 - protein, 9 aa, synthetic construct
GGVGSDSLE

SEQ ID NO: 40023 - protein, 9 aa, synthetic construct
GGVGSDSLL

SEQ ID NO: 40024 - protein, 9 aa, synthetic construct
GGVGSDSLR

SEQ ID NO: 40025 - protein, 9 aa, synthetic construct
GGVGSDSLT

SEQ ID NO: 40026 - protein, 9 aa, synthetic construct
GGVGSDSLY

SEQ ID NO: 40027 - protein, 9 aa, synthetic construct
GGVGSDSMN

SEQ ID NO: 40028 - protein, 9 aa, synthetic construct
GGVGSDSVT

SEQ ID NO: 40029 - protein, 9 aa, synthetic construct
GGVGSDTAD

SEQ ID NO: 40030 - protein, 9 aa, synthetic construct
GGVGSDTAN

SEQ ID NO: 40031 - protein, 9 aa, synthetic construct
GGVGSDRLD

SEQ ID NO: 40032 - protein, 9 aa, synthetic construct
GGVGSDTFK

SEQ ID NO: 40033 - protein, 9 aa, synthetic construct
GGVGSDTID

SEQ ID NO: 40034 - protein, 9 aa, synthetic construct
GGVGSDTIH

SEQ ID NO: 40035 - protein, 9 aa, synthetic construct
GGVGSDTLA

SEQ ID NO: 40036 - protein, 9 aa, synthetic construct
GGVGSDTLF

SEQ ID NO: 40037 - protein, 9 aa, synthetic construct
GGVGSDTLI

SEQ ID NO: 40038 - protein, 9 aa, synthetic construct
GGVGSDTLR

SEQ ID NO: 40039 - protein, 9 aa, synthetic construct
GGVGSDTMD

SEQ ID NO: 40040 - protein, 9 aa, synthetic construct
GGVGSDTMN

SEQ ID NO: 40041 - protein, 9 aa, synthetic construct
GGVGSDTVN

SEQ ID NO: 40042 - protein, 9 aa, synthetic construct
GGVGSDTYR

SEQ ID NO: 40043 - protein, 9 aa, synthetic construct
GGVGSDTYW

SEQ ID NO: 40044 - protein, 9 aa, synthetic construct
GGVGSDVAT

SEQ ID NO: 40045 - protein, 9 aa, synthetic construct
GGVGSDRLS

SEQ ID NO: 40046 - protein, 9 aa, synthetic construct
GGVGSDRIF

SEQ ID NO: 40047 - protein, 9 aa, synthetic construct
GGVGSDFLG

SEQ ID NO: 40048 - protein, 9 aa, synthetic construct
GGVGSDKIY

SEQ ID NO: 40049 - protein, 9 aa, synthetic construct
GGVGSDFLH

SEQ ID NO: 40050 - protein, 9 aa, synthetic construct
GGVGSDFLM

SEQ ID NO: 40051 - protein, 9 aa, synthetic construct
GGVGSDFLT

SEQ ID NO: 40052 - protein, 9 aa, synthetic construct
GGVGSDFVR

SEQ ID NO: 40053 - protein, 9 aa, synthetic construct
GGVGSDGLT

SEQ ID NO: 40054 - protein, 9 aa, synthetic construct
GGVGSDGYV

SEQ ID NO: 40055 - protein, 9 aa, synthetic construct
GGVGSDIAA

SEQ ID NO: 40056 - protein, 9 aa, synthetic construct
GGVGSDIIA

SEQ ID NO: 40057 - protein, 9 aa, synthetic construct
GGVGSDILD

SEQ ID NO: 40058 - protein, 9 aa, synthetic construct
GGVGSDILF

SEQ ID NO: 40059 - protein, 9 aa, synthetic construct
GGVGSDILH

SEQ ID NO: 40060 - protein, 9 aa, synthetic construct
GGVGSDILY

SEQ ID NO: 40061 - protein, 9 aa, synthetic construct
GGVGSDIYV

SEQ ID NO: 40062 - protein, 9 aa, synthetic construct
GGVGSDKLS

SEQ ID NO: 40063 - protein, 9 aa, synthetic construct
GGVGSDRID

SEQ ID NO: 40064 - protein, 9 aa, synthetic construct
GGVGSDKMS

SEQ ID NO: 40065 - protein, 9 aa, synthetic construct
GGVGSDLFA

SEQ ID NO: 40066 - protein, 9 aa, synthetic construct
GGVGSDLIN

SEQ ID NO: 40067 - protein, 9 aa, synthetic construct
GGVGSDLLE

SEQ ID NO: 40068 - protein, 9 aa, synthetic construct
GGVGSDLLI

SEQ ID NO: 40069 - protein, 9 aa, synthetic construct
GGVGSDLLR

SEQ ID NO: 40070 - protein, 9 aa, synthetic construct
GGVGSDMLA

SEQ ID NO: 40071 - protein, 9 aa, synthetic construct
GGVGSDNLT

SEQ ID NO: 40072 - protein, 9 aa, synthetic construct
GGVGSDQLD

SEQ ID NO: 40073 - protein, 9 aa, synthetic construct
GGVGSDQLY

SEQ ID NO: 40074 - protein, 9 aa, synthetic construct
GGVGSDQMF

SEQ ID NO: 40075 - protein, 9 aa, synthetic construct
GGVGSDRAT

SEQ ID NO: 40076 - protein, 9 aa, synthetic construct
GGVGSDRFV

SEQ ID NO: 40077 - protein, 9 aa, synthetic construct
GGWGADVLI

SEQ ID NO: 40078 - protein, 9 aa, synthetic construct
GGWGADYLS

SEQ ID NO: 40079 - protein, 9 aa, synthetic construct
GGWGADYLV

SEQ ID NO: 40080 - protein, 9 aa, synthetic construct
GGWGKDTYV

SEQ ID NO: 40081 - protein, 9 aa, synthetic construct
GGWGNDLII

SEQ ID NO: 40082 - protein, 9 aa, synthetic construct
GGWGNDLIN

SEQ ID NO: 40083 - protein, 9 aa, synthetic construct
GGWGNDLLA

SEQ ID NO: 40084 - protein, 9 aa, synthetic construct
GGWGNDLLL

SEQ ID NO: 40085 - protein, 9 aa, synthetic construct
GGWGNDLVN

SEQ ID NO: 40086 - protein, 9 aa, synthetic construct
GGWGNDQLD

SEQ ID NO: 40087 - protein, 9 aa, synthetic construct
GGWGNDQLL

SEQ ID NO: 40088 - protein, 9 aa, synthetic construct
GGWGNDRID

SEQ ID NO: 40089 - protein, 9 aa, synthetic construct
GGWGNDRIN

SEQ ID NO: 40090 - protein, 9 aa, synthetic construct
GGWGNDRIW

SEQ ID NO: 40091 - protein, 9 aa, synthetic construct
GGWGNDRLE

SEQ ID NO: 40092 - protein, 9 aa, synthetic construct
GGWGNDRLN

SEQ ID NO: 40093 - protein, 9 aa, synthetic construct
GGWGNDSIE

SEQ ID NO: 40094 - protein, 9 aa, synthetic construct
GGWGNDSIL

SEQ ID NO: 40095 - protein, 9 aa, synthetic construct
GGWGNDSIR

SEQ ID NO: 40096 - protein, 9 aa, synthetic construct
GGWGNDSLD

SEQ ID NO: 40097 - protein, 9 aa, synthetic construct
GGWGNDSLK

SEQ ID NO: 40098 - protein, 9 aa, synthetic construct
GGWGNDSLL

SEQ ID NO: 40099 - protein, 9 aa, synthetic construct
GGWGNDSLN

SEQ ID NO: 40100 - protein, 9 aa, synthetic construct
GGWGNDSLT

SEQ ID NO: 40101 - protein, 9 aa, synthetic construct
GGWGNDTFL

SEQ ID NO: 40102 - protein, 9 aa, synthetic construct
GGWGNDTFQ

SEQ ID NO: 40103 - protein, 9 aa, synthetic construct
GGWGNDTIF

SEQ ID NO: 40104 - protein, 9 aa, synthetic construct
GGWGNDTIL

SEQ ID NO: 40105 - protein, 9 aa, synthetic construct
GGWGNDTIW

SEQ ID NO: 40106 - protein, 9 aa, synthetic construct
GGWGNDTLA

SEQ ID NO: 40107 - protein, 9 aa, synthetic construct
GGWGNDTLD

SEQ ID NO: 40108 - protein, 9 aa, synthetic construct
GGWGNDTLG

SEQ ID NO: 40109 - protein, 9 aa, synthetic construct
GGWGNDTMD

SEQ ID NO: 40110 - protein, 9 aa, synthetic construct
GGWGNDKVS

SEQ ID NO: 40111 - protein, 9 aa, synthetic construct
GGWGNDKMY

SEQ ID NO: 40112 - protein, 9 aa, synthetic construct
GGWGNDKLY

SEQ ID NO: 40113 - protein, 9 aa, synthetic construct
GGWGNDGIA

SEQ ID NO: 40114 - protein, 9 aa, synthetic construct
GGWGKDVLT

SEQ ID NO: 40115 - protein, 9 aa, synthetic construct
GGWGLDQYL

SEQ ID NO: 40116 - protein, 9 aa, synthetic construct
GGWGLDTIF

SEQ ID NO: 40117 - protein, 9 aa, synthetic construct
GGWGLDTLS

SEQ ID NO: 40118 - protein, 9 aa, synthetic construct
GGWGLDVVE

SEQ ID NO: 40119 - protein, 9 aa, synthetic construct
GGWGMDTLD

SEQ ID NO: 40120 - protein, 9 aa, synthetic construct
GGWGNDALA

SEQ ID NO: 40121 - protein, 9 aa, synthetic construct
GGWGNDDIN

SEQ ID NO: 40122 - protein, 9 aa, synthetic construct
GGWGNDDIS

SEQ ID NO: 40123 - protein, 9 aa, synthetic construct
GGWGNDEIR

SEQ ID NO: 40124 - protein, 9 aa, synthetic construct
GGWGNDFLA

SEQ ID NO: 40125 - protein, 9 aa, synthetic construct
GGWGNDFLR

SEQ ID NO: 40126 - protein, 9 aa, synthetic construct
GGWGNDFLY

SEQ ID NO: 40127 - protein, 9 aa, synthetic construct
GGWGNDHID

SEQ ID NO: 40128 - protein, 9 aa, synthetic construct
GGWGNDKLF

SEQ ID NO: 40129 - protein, 9 aa, synthetic construct
GGWGNDHIE

SEQ ID NO: 40130 - protein, 9 aa, synthetic construct
GGWGNDHLY

SEQ ID NO: 40131 - protein, 9 aa, synthetic construct
GGWGNDHYI

SEQ ID NO: 40132 - protein, 9 aa, synthetic construct
GGWGNDIFV

SEQ ID NO: 40133 - protein, 9 aa, synthetic construct
GGWGNDILA

SEQ ID NO: 40134 - protein, 9 aa, synthetic construct
GGWGNDILF

SEQ ID NO: 40135 - protein, 9 aa, synthetic construct
GGWGNDILI

SEQ ID NO: 40136 - protein, 9 aa, synthetic construct
GGWGNDILL

SEQ ID NO: 40137 - protein, 9 aa, synthetic construct
GGWGNDILR

SEQ ID NO: 40138 - protein, 9 aa, synthetic construct
GGWGNDIVD

SEQ ID NO: 40139 - protein, 9 aa, synthetic construct
GGWGNDIYN

SEQ ID NO: 40140 - protein, 9 aa, synthetic construct
GGWGNDIYY

SEQ ID NO: 40141 - protein, 9 aa, synthetic construct
GGWGNDKLE

SEQ ID NO: 40142 - protein, 9 aa, synthetic construct
GGWGNDTVV

SEQ ID NO: 40143 - protein, 9 aa, synthetic construct
GGWGNDTVW

SEQ ID NO: 40144 - protein, 9 aa, synthetic construct
GGWGNDTVY

SEQ ID NO: 40145 - protein, 9 aa, synthetic construct
GGWGSDQYL

SEQ ID NO: 40146 - protein, 9 aa, synthetic construct
GGWGRDVFI

SEQ ID NO: 40147 - protein, 9 aa, synthetic construct
GGWGRDVFT

SEQ ID NO: 40148 - protein, 9 aa, synthetic construct
GGWGRDVFY

SEQ ID NO: 40149 - protein, 9 aa, synthetic construct
GGWGRDVLD

SEQ ID NO: 40150 - protein, 9 aa, synthetic construct
GGWGSDALR

SEQ ID NO: 40151 - protein, 9 aa, synthetic construct
GGWGSDLLI

SEQ ID NO: 40152 - protein, 9 aa, synthetic construct
GGWGSDLLN

SEQ ID NO: 40153 - protein, 9 aa, synthetic construct
GGWGSDLLT

SEQ ID NO: 40154 - protein, 9 aa, synthetic construct
GGWGSDLMT

SEQ ID NO: 40155 - protein, 9 aa, synthetic construct
GGWGSDLYS

SEQ ID NO: 40156 - protein, 9 aa, synthetic construct
GGWGSDMLS

SEQ ID NO: 40157 - protein, 9 aa, synthetic construct
GGWGSDNLQ

SEQ ID NO: 40158 - protein, 9 aa, synthetic construct
GGWGSDQMQ

SEQ ID NO: 40159 - protein, 9 aa, synthetic construct
GGWGSDRMF

SEQ ID NO: 40160 - protein, 9 aa, synthetic construct
GGWGRDTVR

SEQ ID NO: 40161 - protein, 9 aa, synthetic construct
GGWGSDTAS

SEQ ID NO: 40162 - protein, 9 aa, synthetic construct
GGWGSDTFV

SEQ ID NO: 40163 - protein, 9 aa, synthetic construct
GGWGSDTID

SEQ ID NO: 40164 - protein, 9 aa, synthetic construct
GGWGSDTLN

SEQ ID NO: 40165 - protein, 9 aa, synthetic construct
GGWGSDVYY

SEQ ID NO: 40166 - protein, 9 aa, synthetic construct
GGWGSDWIS

SEQ ID NO: 40167 - protein, 9 aa, synthetic construct
GGWGSDWLS

SEQ ID NO: 40168 - protein, 9 aa, synthetic construct
GGWGTDAAY

SEQ ID NO: 40169 - protein, 9 aa, synthetic construct
GGWGTDALF

SEQ ID NO: 40170 - protein, 9 aa, synthetic construct
GGWGTDLFR

SEQ ID NO: 40171 - protein, 9 aa, synthetic construct
GGWGTDQVE

SEQ ID NO: 40172 - protein, 9 aa, synthetic construct
GGWGTDRMT

SEQ ID NO: 40173 - protein, 9 aa, synthetic construct
GGWGTDSAY

SEQ ID NO: 40174 - protein, 9 aa, synthetic construct
GGWGRDVFH

SEQ ID NO: 40175 - protein, 9 aa, synthetic construct
GGWGRDTVL

SEQ ID NO: 40176 - protein, 9 aa, synthetic construct
GGWGNDVFV

SEQ ID NO: 40177 - protein, 9 aa, synthetic construct
GGWGQDTLY

SEQ ID NO: 40178 - protein, 9 aa, synthetic construct
GGWGNDVIN

SEQ ID NO: 40179 - protein, 9 aa, synthetic construct
GGWGNDVLH

SEQ ID NO: 40180 - protein, 9 aa, synthetic construct
GGWGNDVLN

SEQ ID NO: 40181 - protein, 9 aa, synthetic construct
GGWGNDVLR

SEQ ID NO: 40182 - protein, 9 aa, synthetic construct
GGWGNDWID

SEQ ID NO: 40183 - protein, 9 aa, synthetic construct
GGWGNDWLY

SEQ ID NO: 40184 - protein, 9 aa, synthetic construct
GGWGNDYID

SEQ ID NO: 40185 - protein, 9 aa, synthetic construct
GGWGNDYIN

SEQ ID NO: 40186 - protein, 9 aa, synthetic construct
GGWGPDRLQ

SEQ ID NO: 40187 - protein, 9 aa, synthetic construct
GGWGQDILN

SEQ ID NO: 40188 - protein, 9 aa, synthetic construct
GGWGQDLLL

SEQ ID NO: 40189 - protein, 9 aa, synthetic construct
GGWGQDTAS

SEQ ID NO: 40190 - protein, 9 aa, synthetic construct
GGWGQDTLT

SEQ ID NO: 40191 - protein, 9 aa, synthetic construct
GGWGQDYLD

SEQ ID NO: 40192 - protein, 9 aa, synthetic construct
GGWGRDTVK

SEQ ID NO: 40193 - protein, 9 aa, synthetic construct
GGWGRDDLK

SEQ ID NO: 40194 - protein, 9 aa, synthetic construct
GGWGRDIFT

SEQ ID NO: 40195 - protein, 9 aa, synthetic construct
GGWGRDKAN

SEQ ID NO: 40196 - protein, 9 aa, synthetic construct
GGWGRDLLH

SEQ ID NO: 40197 - protein, 9 aa, synthetic construct
GGWGRDMLF

SEQ ID NO: 40198 - protein, 9 aa, synthetic construct
GGWGRDQFV

SEQ ID NO: 40199 - protein, 9 aa, synthetic construct
GGWGRDRIW

SEQ ID NO: 40200 - protein, 9 aa, synthetic construct
GGWGRDSLE

SEQ ID NO: 40201 - protein, 9 aa, synthetic construct
GGWGRDSLK

SEQ ID NO: 40202 - protein, 9 aa, synthetic construct
GGWGRDTFV

SEQ ID NO: 40203 - protein, 9 aa, synthetic construct
GGWGRDTLF

SEQ ID NO: 40204 - protein, 9 aa, synthetic construct
GGWGRDTLI

SEQ ID NO: 40205 - protein, 9 aa, synthetic construct
GGWGRDTLL

SEQ ID NO: 40206 - protein, 9 aa, synthetic construct
GGWGKDVLS

SEQ ID NO: 40207 - protein, 9 aa, synthetic construct
GGWGKDTLN

SEQ ID NO: 40208 - protein, 9 aa, synthetic construct
GGWGDDAIW

SEQ ID NO: 40209 - protein, 9 aa, synthetic construct
GGWGKDTLI

SEQ ID NO: 40210 - protein, 9 aa, synthetic construct
GGWGDDRIV

SEQ ID NO: 40211 - protein, 9 aa, synthetic construct
GGWGDDRLF

SEQ ID NO: 40212 - protein, 9 aa, synthetic construct
GGWGDDRLI

SEQ ID NO: 40213 - protein, 9 aa, synthetic construct
GGWGDDRLV

SEQ ID NO: 40214 - protein, 9 aa, synthetic construct
GGWGDDRLW

SEQ ID NO: 40215 - protein, 9 aa, synthetic construct
GGWGDDRLY

SEQ ID NO: 40216 - protein, 9 aa, synthetic construct
GGWGDDRMF

SEQ ID NO: 40217 - protein, 9 aa, synthetic construct
GGWGDDRVF

SEQ ID NO: 40218 - protein, 9 aa, synthetic construct
GGWGDDSLT

SEQ ID NO: 40219 - protein, 9 aa, synthetic construct
GGWGDDSVD

SEQ ID NO: 40220 - protein, 9 aa, synthetic construct
GGWGDDTAT

SEQ ID NO: 40221 - protein, 9 aa, synthetic construct
GGWGDDTAV

SEQ ID NO: 40222 - protein, 9 aa, synthetic construct
GGWGDDTFY

SEQ ID NO: 40223 - protein, 9 aa, synthetic construct
GGWGDDTIE

SEQ ID NO: 40224 - protein, 9 aa, synthetic construct
GGWGDDTIH

SEQ ID NO: 40225 - protein, 9 aa, synthetic construct
GGWGDDTII

SEQ ID NO: 40226 - protein, 9 aa, synthetic construct
GGWGDDTLG

SEQ ID NO: 40227 - protein, 9 aa, synthetic construct
GGWGDDTLH

SEQ ID NO: 40228 - protein, 9 aa, synthetic construct
GGWGDDTLM

SEQ ID NO: 40229 - protein, 9 aa, synthetic construct
GGWGDDTLQ

SEQ ID NO: 40230 - protein, 9 aa, synthetic construct
GGWGDDTLR

SEQ ID NO: 40231 - protein, 9 aa, synthetic construct
GGWGDDTLV

SEQ ID NO: 40232 - protein, 9 aa, synthetic construct
GGWGDDTMT

SEQ ID NO: 40233 - protein, 9 aa, synthetic construct
GGWGDDTMY

SEQ ID NO: 40234 - protein, 9 aa, synthetic construct
GGWGDDTVN

SEQ ID NO: 40235 - protein, 9 aa, synthetic construct
GGWGDDTVS

SEQ ID NO: 40236 - protein, 9 aa, synthetic construct
GGWGDDTYV

SEQ ID NO: 40237 - protein, 9 aa, synthetic construct
GGWGDDVFL

SEQ ID NO: 40238 - protein, 9 aa, synthetic construct
GGWGDDVFY

SEQ ID NO: 40239 - protein, 9 aa, synthetic construct
GGWGDDRFS

SEQ ID NO: 40240 - protein, 9 aa, synthetic construct
GGWGDDQLY

SEQ ID NO: 40241 - protein, 9 aa, synthetic construct
GGWGDDQAF

SEQ ID NO: 40242 - protein, 9 aa, synthetic construct
GGWGDDILR

SEQ ID NO: 40243 - protein, 9 aa, synthetic construct
GGWGDDALT

SEQ ID NO: 40244 - protein, 9 aa, synthetic construct
GGWGDDDIN

SEQ ID NO: 40245 - protein, 9 aa, synthetic construct
GGWGDDEID

SEQ ID NO: 40246 - protein, 9 aa, synthetic construct
GGWGDDEIH

SEQ ID NO: 40247 - protein, 9 aa, synthetic construct
GGWGDDELT

SEQ ID NO: 40248 - protein, 9 aa, synthetic construct
GGWGDDEML

SEQ ID NO: 40249 - protein, 9 aa, synthetic construct
GGWGDDFIN

SEQ ID NO: 40250 - protein, 9 aa, synthetic construct
GGWGDDFMA

SEQ ID NO: 40251 - protein, 9 aa, synthetic construct
GGWGDDHLY

SEQ ID NO: 40252 - protein, 9 aa, synthetic construct
GGWGDDIID

SEQ ID NO: 40253 - protein, 9 aa, synthetic construct
GGWGDDIIL

SEQ ID NO: 40254 - protein, 9 aa, synthetic construct
GGWGDDILI

SEQ ID NO: 40255 - protein, 9 aa, synthetic construct
GGWGDDILN

SEQ ID NO: 40256 - protein, 9 aa, synthetic construct
GGWGDDILS

SEQ ID NO: 40257 - protein, 9 aa, synthetic construct
GGWGDDMMS

SEQ ID NO: 40258 - protein, 9 aa, synthetic construct
GGWGDDILV

SEQ ID NO: 40259 - protein, 9 aa, synthetic construct
GGWGDDIVA

SEQ ID NO: 40260 - protein, 9 aa, synthetic construct
GGWGDDKLD

SEQ ID NO: 40261 - protein, 9 aa, synthetic construct
GGWGDDKLM

SEQ ID NO: 40262 - protein, 9 aa, synthetic construct
GGWGDDKLW

SEQ ID NO: 40263 - protein, 9 aa, synthetic construct
GGWGDDLAV

SEQ ID NO: 40264 - protein, 9 aa, synthetic construct
GGWGDDLIG

SEQ ID NO: 40265 - protein, 9 aa, synthetic construct
GGWGDDLIN

SEQ ID NO: 40266 - protein, 9 aa, synthetic construct
GGWGDDLLF

SEQ ID NO: 40267 - protein, 9 aa, synthetic construct
GGWGDDLLV

SEQ ID NO: 40268 - protein, 9 aa, synthetic construct
GGWGDDLVR

SEQ ID NO: 40269 - protein, 9 aa, synthetic construct
GGWGDDLVV

SEQ ID NO: 40270 - protein, 9 aa, synthetic construct
GGWGDDMLN

SEQ ID NO: 40271 - protein, 9 aa, synthetic construct
GGWGDDVII

SEQ ID NO: 40272 - protein, 9 aa, synthetic construct
GGWGDDVLL

SEQ ID NO: 40273 - protein, 9 aa, synthetic construct
GGWGDDVLN

SEQ ID NO: 40274 - protein, 9 aa, synthetic construct
GGWGHDTLY

SEQ ID NO: 40275 - protein, 9 aa, synthetic construct
GGWGHDAAW

SEQ ID NO: 40276 - protein, 9 aa, synthetic construct
GGWGHDALH

SEQ ID NO: 40277 - protein, 9 aa, synthetic construct
GGWGHDELK

SEQ ID NO: 40278 - protein, 9 aa, synthetic construct
GGWGHDHLD

SEQ ID NO: 40279 - protein, 9 aa, synthetic construct
GGWGHDILN

SEQ ID NO: 40280 - protein, 9 aa, synthetic construct
GGWGHDLII

SEQ ID NO: 40281 - protein, 9 aa, synthetic construct
GGWGHDMIA

SEQ ID NO: 40282 - protein, 9 aa, synthetic construct
GGWGHDQLN

SEQ ID NO: 40283 - protein, 9 aa, synthetic construct
GGWGHDRLD

SEQ ID NO: 40284 - protein, 9 aa, synthetic construct
GGWGHDRLF

SEQ ID NO: 40285 - protein, 9 aa, synthetic construct
GGWGHDRLT

SEQ ID NO: 40286 - protein, 9 aa, synthetic construct
GGWGHDTII

SEQ ID NO: 40287 - protein, 9 aa, synthetic construct
GGWGHDTLH

SEQ ID NO: 40288 - protein, 9 aa, synthetic construct
GGWGHDTVK

SEQ ID NO: 40289 - protein, 9 aa, synthetic construct
GGWGGDTLY

SEQ ID NO: 40290 - protein, 9 aa, synthetic construct
GGWGHDVLA

SEQ ID NO: 40291 - protein, 9 aa, synthetic construct
GGWGHDVLI

SEQ ID NO: 40292 - protein, 9 aa, synthetic construct
GGWGHDVLT

SEQ ID NO: 40293 - protein, 9 aa, synthetic construct
GGWGHDVMN

SEQ ID NO: 40294 - protein, 9 aa, synthetic construct
GGWGIDSIT

SEQ ID NO: 40295 - protein, 9 aa, synthetic construct
GGWGIDSLN

SEQ ID NO: 40296 - protein, 9 aa, synthetic construct
GGWGKDAFI

SEQ ID NO: 40297 - protein, 9 aa, synthetic construct
GGWGKDIFT

SEQ ID NO: 40298 - protein, 9 aa, synthetic construct
GGWGKDILS

SEQ ID NO: 40299 - protein, 9 aa, synthetic construct
GGWGKDLLN

SEQ ID NO: 40300 - protein, 9 aa, synthetic construct
GGWGKDSFV

SEQ ID NO: 40301 - protein, 9 aa, synthetic construct
GGWGKDTIT

SEQ ID NO: 40302 - protein, 9 aa, synthetic construct
GGWGKDTIY

SEQ ID NO: 40303 - protein, 9 aa, synthetic construct
GGWGGDTYL

SEQ ID NO: 40304 - protein, 9 aa, synthetic construct
GGWGGDTII

SEQ ID NO: 40305 - protein, 9 aa, synthetic construct
GGWGDDVLS

SEQ ID NO: 40306 - protein, 9 aa, synthetic construct
GGWGEDILY

SEQ ID NO: 40307 - protein, 9 aa, synthetic construct
GGWGDDVLV

SEQ ID NO: 40308 - protein, 9 aa, synthetic construct
GGWGDDVLW

SEQ ID NO: 40309 - protein, 9 aa, synthetic construct
GGWGDDVML

SEQ ID NO: 40310 - protein, 9 aa, synthetic construct
GGWGDDVVS

SEQ ID NO: 40311 - protein, 9 aa, synthetic construct
GGWGDDVYA

SEQ ID NO: 40312 - protein, 9 aa, synthetic construct
GGWGDDWIM

SEQ ID NO: 40313 - protein, 9 aa, synthetic construct
GGWGDDWIS

SEQ ID NO: 40314 - protein, 9 aa, synthetic construct
GGWGDDWLE

SEQ ID NO: 40315 - protein, 9 aa, synthetic construct
GGWGDDYIE

SEQ ID NO: 40316 - protein, 9 aa, synthetic construct
GGWGDDYIH

SEQ ID NO: 40317 - protein, 9 aa, synthetic construct
GGWGDDYLV

SEQ ID NO: 40318 - protein, 9 aa, synthetic construct
GGWGEDDLF

SEQ ID NO: 40319 - protein, 9 aa, synthetic construct
GGWGEDILL

SEQ ID NO: 40320 - protein, 9 aa, synthetic construct
GGWGEDMIV

SEQ ID NO: 40321 - protein, 9 aa, synthetic construct
GGWGGDSMV

SEQ ID NO: 40322 - protein, 9 aa, synthetic construct
GGWGEDQLY

SEQ ID NO: 40323 - protein, 9 aa, synthetic construct
GGWGEDSLY

SEQ ID NO: 40324 - protein, 9 aa, synthetic construct
GGWGEDTIR

SEQ ID NO: 40325 - protein, 9 aa, synthetic construct
GGWGEDTLS

SEQ ID NO: 40326 - protein, 9 aa, synthetic construct
GGWGEDTLV

SEQ ID NO: 40327 - protein, 9 aa, synthetic construct
GGWGEDVFA

SEQ ID NO: 40328 - protein, 9 aa, synthetic construct
GGWGFDIIY

SEQ ID NO: 40329 - protein, 9 aa, synthetic construct
GGWGFDTAS

SEQ ID NO: 40330 - protein, 9 aa, synthetic construct
GGWGFDTVS

SEQ ID NO: 40331 - protein, 9 aa, synthetic construct
GGWGFDWIS

SEQ ID NO: 40332 - protein, 9 aa, synthetic construct
GGWGGDMLS

SEQ ID NO: 40333 - protein, 9 aa, synthetic construct
GGWGGDQFI

SEQ ID NO: 40334 - protein, 9 aa, synthetic construct
GGWGGDRIF

SEQ ID NO: 40335 - protein, 9 aa, synthetic construct
GGTGSDKIY

SEQ ID NO: 40336 - protein, 9 aa, synthetic construct
GGTGSDKID

SEQ ID NO: 40337 - protein, 9 aa, synthetic construct
GGTGSDKFV

SEQ ID NO: 40338 - protein, 9 aa, synthetic construct
GGTGADWMT

SEQ ID NO: 40339 - protein, 9 aa, synthetic construct
GGTGADTFE

SEQ ID NO: 40340 - protein, 9 aa, synthetic construct
GGTGADTFM

SEQ ID NO: 40341 - protein, 9 aa, synthetic construct
GGTGADTFQ

SEQ ID NO: 40342 - protein, 9 aa, synthetic construct
GGTGADTIQ

SEQ ID NO: 40343 - protein, 9 aa, synthetic construct
GGTGADTVI

SEQ ID NO: 40344 - protein, 9 aa, synthetic construct
GGTGADTVK

SEQ ID NO: 40345 - protein, 9 aa, synthetic construct
GGTGADTVR

SEQ ID NO: 40346 - protein, 9 aa, synthetic construct
GGTGADTVT

SEQ ID NO: 40347 - protein, 9 aa, synthetic construct
GGTGADTVV

SEQ ID NO: 40348 - protein, 9 aa, synthetic construct
GGTGADTVY

SEQ ID NO: 40349 - protein, 9 aa, synthetic construct
GGTGADTYE

SEQ ID NO: 40350 - protein, 9 aa, synthetic construct
GGTGADTYI

SEQ ID NO: 40351 - protein, 9 aa, synthetic construct
GGTGADTYN

SEQ ID NO: 40352 - protein, 9 aa, synthetic construct
GGTGADVFD

SEQ ID NO: 40353 - protein, 9 aa, synthetic construct
GGTGADVFN

SEQ ID NO: 40354 - protein, 9 aa, synthetic construct
GGTGADVFQ

SEQ ID NO: 40355 - protein, 9 aa, synthetic construct
GGTGADVFS

SEQ ID NO: 40356 - protein, 9 aa, synthetic construct
GGTGADVIV

SEQ ID NO: 40357 - protein, 9 aa, synthetic construct
GGTGADVIY

SEQ ID NO: 40358 - protein, 9 aa, synthetic construct
GGTGADVLW

SEQ ID NO: 40359 - protein, 9 aa, synthetic construct
GGTGADVML

SEQ ID NO: 40360 - protein, 9 aa, synthetic construct
GGTGADVVA

SEQ ID NO: 40361 - protein, 9 aa, synthetic construct
GGTGADVVL

SEQ ID NO: 40362 - protein, 9 aa, synthetic construct
GGTGADWAS

SEQ ID NO: 40363 - protein, 9 aa, synthetic construct
GGTGADWIE

SEQ ID NO: 40364 - protein, 9 aa, synthetic construct
GGTGADWLE

SEQ ID NO: 40365 - protein, 9 aa, synthetic construct
GGTGADWLH

SEQ ID NO: 40366 - protein, 9 aa, synthetic construct
GGTGADWLI

SEQ ID NO: 40367 - protein, 9 aa, synthetic construct
GGTGADWLL

SEQ ID NO: 40368 - protein, 9 aa, synthetic construct
GGTGADSVY

SEQ ID NO: 40369 - protein, 9 aa, synthetic construct
GGTGADSVS

SEQ ID NO: 40370 - protein, 9 aa, synthetic construct
GGTGADSVL

SEQ ID NO: 40371 - protein, 9 aa, synthetic construct
GGTGADRVS

SEQ ID NO: 40372 - protein, 9 aa, synthetic construct
GGTGADRFT

SEQ ID NO: 40373 - protein, 9 aa, synthetic construct
GGTGADRFY

SEQ ID NO: 40374 - protein, 9 aa, synthetic construct
GGTGADRIH

SEQ ID NO: 40375 - protein, 9 aa, synthetic construct
GGTGADRIL

SEQ ID NO: 40376 - protein, 9 aa, synthetic construct
GGTGADRIN

SEQ ID NO: 40377 - protein, 9 aa, synthetic construct
GGTGADRLM

SEQ ID NO: 40378 - protein, 9 aa, synthetic construct
GGTGADRLP

SEQ ID NO: 40379 - protein, 9 aa, synthetic construct
GGTGADRMD

SEQ ID NO: 40380 - protein, 9 aa, synthetic construct
GGTGADRMN

SEQ ID NO: 40381 - protein, 9 aa, synthetic construct
GGTGADRMR

SEQ ID NO: 40382 - protein, 9 aa, synthetic construct
GGTGADRMW

SEQ ID NO: 40383 - protein, 9 aa, synthetic construct
GGTGADRVA

SEQ ID NO: 40384 - protein, 9 aa, synthetic construct
GGTGADRVN

SEQ ID NO: 40385 - protein, 9 aa, synthetic construct
GGTGADSFF

SEQ ID NO: 40386 - protein, 9 aa, synthetic construct
GGTGADSVE

SEQ ID NO: 40387 - protein, 9 aa, synthetic construct
GGTGADSFH

SEQ ID NO: 40388 - protein, 9 aa, synthetic construct
GGTGADSFI

SEQ ID NO: 40389 - protein, 9 aa, synthetic construct
GGTGADSIA

SEQ ID NO: 40390 - protein, 9 aa, synthetic construct
GGTGADSIG

SEQ ID NO: 40391 - protein, 9 aa, synthetic construct
GGTGADSII

SEQ ID NO: 40392 - protein, 9 aa, synthetic construct
GGTGADSLG

SEQ ID NO: 40393 - protein, 9 aa, synthetic construct
GGTGADSLQ

SEQ ID NO: 40394 - protein, 9 aa, synthetic construct
GGTGADSLR

SEQ ID NO: 40395 - protein, 9 aa, synthetic construct
GGTGADSMD

SEQ ID NO: 40396 - protein, 9 aa, synthetic construct
GGTGADSME

SEQ ID NO: 40397 - protein, 9 aa, synthetic construct
GGTGADSMF

SEQ ID NO: 40398 - protein, 9 aa, synthetic construct
GGTGADSMI

SEQ ID NO: 40399 - protein, 9 aa, synthetic construct
GGTGADSMW

SEQ ID NO: 40400 - protein, 9 aa, synthetic construct
GGTGADWLS

SEQ ID NO: 40401 - protein, 9 aa, synthetic construct
GGTGADWVA

SEQ ID NO: 40402 - protein, 9 aa, synthetic construct
GGTGDDGYI

SEQ ID NO: 40403 - protein, 9 aa, synthetic construct
GGTGADYIV

SEQ ID NO: 40404 - protein, 9 aa, synthetic construct
GGTGDDDMR

SEQ ID NO: 40405 - protein, 9 aa, synthetic construct
GGTGDDDMS

SEQ ID NO: 40406 - protein, 9 aa, synthetic construct
GGTGDDDMV

SEQ ID NO: 40407 - protein, 9 aa, synthetic construct
GGTGDDEID

SEQ ID NO: 40408 - protein, 9 aa, synthetic construct
GGTGDDEIY

SEQ ID NO: 40409 - protein, 9 aa, synthetic construct
GGTGDDELG

SEQ ID NO: 40410 - protein, 9 aa, synthetic construct
GGTGDDELK

SEQ ID NO: 40411 - protein, 9 aa, synthetic construct
GGTGDDELR

SEQ ID NO: 40412 - protein, 9 aa, synthetic construct
GGTGDDELT

SEQ ID NO: 40413 - protein, 9 aa, synthetic construct
GGTGDDELW

SEQ ID NO: 40414 - protein, 9 aa, synthetic construct
GGTGDDEYI

SEQ ID NO: 40415 - protein, 9 aa, synthetic construct
GGTGDDFAE

SEQ ID NO: 40416 - protein, 9 aa, synthetic construct
GGTGDDFAV

SEQ ID NO: 40417 - protein, 9 aa, synthetic construct
GGTGDDFFR

SEQ ID NO: 40418 - protein, 9 aa, synthetic construct
GGTGDDFIA

SEQ ID NO: 40419 - protein, 9 aa, synthetic construct
GGTGDDFIS

SEQ ID NO: 40420 - protein, 9 aa, synthetic construct
GGTGDDFIY

SEQ ID NO: 40421 - protein, 9 aa, synthetic construct
GGTGDDFLH

SEQ ID NO: 40422 - protein, 9 aa, synthetic construct
GGTGDDFLI

SEQ ID NO: 40423 - protein, 9 aa, synthetic construct
GGTGDDFLQ

SEQ ID NO: 40424 - protein, 9 aa, synthetic construct
GGTGDDFMG

SEQ ID NO: 40425 - protein, 9 aa, synthetic construct
GGTGDDFVL

SEQ ID NO: 40426 - protein, 9 aa, synthetic construct
GGTGDDFVQ

SEQ ID NO: 40427 - protein, 9 aa, synthetic construct
GGTGDDFYS

SEQ ID NO: 40428 - protein, 9 aa, synthetic construct
GGTGDDGIW

SEQ ID NO: 40429 - protein, 9 aa, synthetic construct
GGTGDDGLA

SEQ ID NO: 40430 - protein, 9 aa, synthetic construct
GGTGDDGLI

SEQ ID NO: 40431 - protein, 9 aa, synthetic construct
GGTGDDGMK

SEQ ID NO: 40432 - protein, 9 aa, synthetic construct
GGTGDDGVI

SEQ ID NO: 40433 - protein, 9 aa, synthetic construct
GGTGDDDML

SEQ ID NO: 40434 - protein, 9 aa, synthetic construct
GGTGDDDME

SEQ ID NO: 40435 - protein, 9 aa, synthetic construct
GGTGDDDLW

SEQ ID NO: 40436 - protein, 9 aa, synthetic construct
GGTGDDALA

SEQ ID NO: 40437 - protein, 9 aa, synthetic construct
GGTGADYLL

SEQ ID NO: 40438 - protein, 9 aa, synthetic construct
GGTGADYLW

SEQ ID NO: 40439 - protein, 9 aa, synthetic construct
GGTGADYMV

SEQ ID NO: 40440 - protein, 9 aa, synthetic construct
GGTGADYVD

SEQ ID NO: 40441 - protein, 9 aa, synthetic construct
GGTGCDRLR

SEQ ID NO: 40442 - protein, 9 aa, synthetic construct
GGTGCDTYV

SEQ ID NO: 40443 - protein, 9 aa, synthetic construct
GGTGCDYIY

SEQ ID NO: 40444 - protein, 9 aa, synthetic construct
GGTGDDAIF

SEQ ID NO: 40445 - protein, 9 aa, synthetic construct
GGTGDDAIG

SEQ ID NO: 40446 - protein, 9 aa, synthetic construct
GGTGDDAIM

SEQ ID NO: 40447 - protein, 9 aa, synthetic construct
GGTGDDAIN

SEQ ID NO: 40448 - protein, 9 aa, synthetic construct
GGTGDDAIT

SEQ ID NO: 40449 - protein, 9 aa, synthetic construct
GGTGDDAIY

SEQ ID NO: 40450 - protein, 9 aa, synthetic construct
GGTGDDALI

SEQ ID NO: 40451 - protein, 9 aa, synthetic construct
GGTGDDDLQ

SEQ ID NO: 40452 - protein, 9 aa, synthetic construct
GGTGDDALM

SEQ ID NO: 40453 - protein, 9 aa, synthetic construct
GGTGDDALN

SEQ ID NO: 40454 - protein, 9 aa, synthetic construct
GGTGDDALV

SEQ ID NO: 40455 - protein, 9 aa, synthetic construct
GGTGDDAMT

SEQ ID NO: 40456 - protein, 9 aa, synthetic construct
GGTGDDAVT

SEQ ID NO: 40457 - protein, 9 aa, synthetic construct
GGTGDDCLD

SEQ ID NO: 40458 - protein, 9 aa, synthetic construct
GGTGDDDIM

SEQ ID NO: 40459 - protein, 9 aa, synthetic construct
GGTGDDDIN

SEQ ID NO: 40460 - protein, 9 aa, synthetic construct
GGTGDDDIQ

SEQ ID NO: 40461 - protein, 9 aa, synthetic construct
GGTGDDDIR

SEQ ID NO: 40462 - protein, 9 aa, synthetic construct
GGTGDDDIY

SEQ ID NO: 40463 - protein, 9 aa, synthetic construct
GGTGDDDLA

SEQ ID NO: 40464 - protein, 9 aa, synthetic construct
GGTGDDDLI

SEQ ID NO: 40465 - protein, 9 aa, synthetic construct
GGTGADRFN

SEQ ID NO: 40466 - protein, 9 aa, synthetic construct
GGTGADRFK

SEQ ID NO: 40467 - protein, 9 aa, synthetic construct
GGTGADQMW

SEQ ID NO: 40468 - protein, 9 aa, synthetic construct
GGTGADQMT

SEQ ID NO: 40469 - protein, 9 aa, synthetic construct
GGTGADFIE

SEQ ID NO: 40470 - protein, 9 aa, synthetic construct
GGTGADFIS

SEQ ID NO: 40471 - protein, 9 aa, synthetic construct
GGTGADFLH

SEQ ID NO: 40472 - protein, 9 aa, synthetic construct
GGTGADFLI

SEQ ID NO: 40473 - protein, 9 aa, synthetic construct
GGTGADFLN

SEQ ID NO: 40474 - protein, 9 aa, synthetic construct
GGTGADFLS

SEQ ID NO: 40475 - protein, 9 aa, synthetic construct
GGTGADFMD

SEQ ID NO: 40476 - protein, 9 aa, synthetic construct
GGTGADFMF

SEQ ID NO: 40477 - protein, 9 aa, synthetic construct
GGTGADFMV

SEQ ID NO: 40478 - protein, 9 aa, synthetic construct
GGTGADFVD

SEQ ID NO: 40479 - protein, 9 aa, synthetic construct
GGTGADGLS

SEQ ID NO: 40480 - protein, 9 aa, synthetic construct
GGTGADGMF

SEQ ID NO: 40481 - protein, 9 aa, synthetic construct
GGTGADHAE

SEQ ID NO: 40482 - protein, 9 aa, synthetic construct
GGTGADHFD

SEQ ID NO: 40483 - protein, 9 aa, synthetic construct
GGTGADHIN

SEQ ID NO: 40484 - protein, 9 aa, synthetic construct
GGTGADHLF

SEQ ID NO: 40485 - protein, 9 aa, synthetic construct
GGTGADHLS

SEQ ID NO: 40486 - protein, 9 aa, synthetic construct
GGTGADHLT

SEQ ID NO: 40487 - protein, 9 aa, synthetic construct
GGTGADHLV

SEQ ID NO: 40488 - protein, 9 aa, synthetic construct
GGTGADHLY

SEQ ID NO: 40489 - protein, 9 aa, synthetic construct
GGTGADHMD

SEQ ID NO: 40490 - protein, 9 aa, synthetic construct
GGTGADHMS

SEQ ID NO: 40491 - protein, 9 aa, synthetic construct
GGTGADHYL

SEQ ID NO: 40492 - protein, 9 aa, synthetic construct
GGTGADIFE

SEQ ID NO: 40493 - protein, 9 aa, synthetic construct
GGTGADIFF

SEQ ID NO: 40494 - protein, 9 aa, synthetic construct
GGTGADIFI

SEQ ID NO: 40495 - protein, 9 aa, synthetic construct
GGTGADIIE

SEQ ID NO: 40496 - protein, 9 aa, synthetic construct
GGTGADIII

SEQ ID NO: 40497 - protein, 9 aa, synthetic construct
GGTGADIIL

SEQ ID NO: 40498 - protein, 9 aa, synthetic construct
GGTGADFFN

SEQ ID NO: 40499 - protein, 9 aa, synthetic construct
GGTGADFAR

SEQ ID NO: 40500 - protein, 9 aa, synthetic construct
GGTGADEYY

SEQ ID NO: 40501 - protein, 9 aa, synthetic construct
GGTGADDLA

SEQ ID NO: 40502 - protein, 9 aa, synthetic construct
GGTGADALV

SEQ ID NO: 40503 - protein, 9 aa, synthetic construct
GGTGADALW

SEQ ID NO: 40504 - protein, 9 aa, synthetic construct
GGTGADAMF

SEQ ID NO: 40505 - protein, 9 aa, synthetic construct
GGTGADAMK

SEQ ID NO: 40506 - protein, 9 aa, synthetic construct
GGTGADAMV

SEQ ID NO: 40507 - protein, 9 aa, synthetic construct
GGTGADAMY

SEQ ID NO: 40508 - protein, 9 aa, synthetic construct
GGTGADAVH

SEQ ID NO: 40509 - protein, 9 aa, synthetic construct
GGTGADAYS

SEQ ID NO: 40510 - protein, 9 aa, synthetic construct
GGTGADDFD

SEQ ID NO: 40511 - protein, 9 aa, synthetic construct
GGTGADDFV

SEQ ID NO: 40512 - protein, 9 aa, synthetic construct
GGTGADDIF

SEQ ID NO: 40513 - protein, 9 aa, synthetic construct
GGTGADDIL

SEQ ID NO: 40514 - protein, 9 aa, synthetic construct
GGTGADDIR

SEQ ID NO: 40515 - protein, 9 aa, synthetic construct
GGTGADDLF

SEQ ID NO: 40516 - protein, 9 aa, synthetic construct
GGTGADEMT

SEQ ID NO: 40517 - protein, 9 aa, synthetic construct
GGTGADDLH

SEQ ID NO: 40518 - protein, 9 aa, synthetic construct
GGTGADDML

SEQ ID NO: 40519 - protein, 9 aa, synthetic construct
GGTGADDMN

SEQ ID NO: 40520 - protein, 9 aa, synthetic construct
GGTGADDMQ

SEQ ID NO: 40521 - protein, 9 aa, synthetic construct
GGTGADDMS

SEQ ID NO: 40522 - protein, 9 aa, synthetic construct
GGTGADDYV

SEQ ID NO: 40523 - protein, 9 aa, synthetic construct
GGTGADEFR

SEQ ID NO: 40524 - protein, 9 aa, synthetic construct
GGTGADEIL

SEQ ID NO: 40525 - protein, 9 aa, synthetic construct
GGTGADEIS

SEQ ID NO: 40526 - protein, 9 aa, synthetic construct
GGTGADEIY

SEQ ID NO: 40527 - protein, 9 aa, synthetic construct
GGTGADELQ

SEQ ID NO: 40528 - protein, 9 aa, synthetic construct
GGTGADELR

SEQ ID NO: 40529 - protein, 9 aa, synthetic construct
GGTGADEME

SEQ ID NO: 40530 - protein, 9 aa, synthetic construct
GGTGADILE

SEQ ID NO: 40531 - protein, 9 aa, synthetic construct
GGTGADILY

SEQ ID NO: 40532 - protein, 9 aa, synthetic construct
GGTGADIMF

SEQ ID NO: 40533 - protein, 9 aa, synthetic construct
GGTGADQAF

SEQ ID NO: 40534 - protein, 9 aa, synthetic construct
GGTGADNFI

SEQ ID NO: 40535 - protein, 9 aa, synthetic construct
GGTGADNFK

SEQ ID NO: 40536 - protein, 9 aa, synthetic construct
GGTGADNFN

SEQ ID NO: 40537 - protein, 9 aa, synthetic construct
GGTGADNFY

SEQ ID NO: 40538 - protein, 9 aa, synthetic construct
GGTGADNIV

SEQ ID NO: 40539 - protein, 9 aa, synthetic construct
GGTGADNLG

SEQ ID NO: 40540 - protein, 9 aa, synthetic construct
GGTGADNLK

SEQ ID NO: 40541 - protein, 9 aa, synthetic construct
GGTGADNLS

SEQ ID NO: 40542 - protein, 9 aa, synthetic construct
GGTGADNLY

SEQ ID NO: 40543 - protein, 9 aa, synthetic construct
GGTGADNMF

SEQ ID NO: 40544 - protein, 9 aa, synthetic construct
GGTGADNMI

SEQ ID NO: 40545 - protein, 9 aa, synthetic construct
GGTGADNMV

SEQ ID NO: 40546 - protein, 9 aa, synthetic construct
GGTGADNYL

SEQ ID NO: 40547 - protein, 9 aa, synthetic construct
GGTGADQFD

SEQ ID NO: 40548 - protein, 9 aa, synthetic construct
GGTGADMMT

SEQ ID NO: 40549 - protein, 9 aa, synthetic construct
GGTGADQFI

SEQ ID NO: 40550 - protein, 9 aa, synthetic construct
GGTGADQFY

SEQ ID NO: 40551 - protein, 9 aa, synthetic construct
GGTGADQIF

SEQ ID NO: 40552 - protein, 9 aa, synthetic construct
GGTGADQIY

SEQ ID NO: 40553 - protein, 9 aa, synthetic construct
GGTGADQLA

SEQ ID NO: 40554 - protein, 9 aa, synthetic construct
GGTGADQLL

SEQ ID NO: 40555 - protein, 9 aa, synthetic construct
GGTGADQLN

SEQ ID NO: 40556 - protein, 9 aa, synthetic construct
GGTGADQLS

SEQ ID NO: 40557 - protein, 9 aa, synthetic construct
GGTGADQLV

SEQ ID NO: 40558 - protein, 9 aa, synthetic construct
GGTGADQMF

SEQ ID NO: 40559 - protein, 9 aa, synthetic construct
GGTGADQML

SEQ ID NO: 40560 - protein, 9 aa, synthetic construct
GGTGADQMR

SEQ ID NO: 40561 - protein, 9 aa, synthetic construct
GGTGADQMS

SEQ ID NO: 40562 - protein, 9 aa, synthetic construct
GGTGADMMV

SEQ ID NO: 40563 - protein, 9 aa, synthetic construct
GGTGADMMD

SEQ ID NO: 40564 - protein, 9 aa, synthetic construct
GGTGADIMH

SEQ ID NO: 40565 - protein, 9 aa, synthetic construct
GGTGADKME

SEQ ID NO: 40566 - protein, 9 aa, synthetic construct
GGTGADIMQ

SEQ ID NO: 40567 - protein, 9 aa, synthetic construct
GGTGADIMY

SEQ ID NO: 40568 - protein, 9 aa, synthetic construct
GGTGADIVA

SEQ ID NO: 40569 - protein, 9 aa, synthetic construct
GGTGADIVK

SEQ ID NO: 40570 - protein, 9 aa, synthetic construct
GGTGADIVR

SEQ ID NO: 40571 - protein, 9 aa, synthetic construct
GGTGADIVV

SEQ ID NO: 40572 - protein, 9 aa, synthetic construct
GGTGADIVY

SEQ ID NO: 40573 - protein, 9 aa, synthetic construct
GGTGADIYA

SEQ ID NO: 40574 - protein, 9 aa, synthetic construct
GGTGADIYY

SEQ ID NO: 40575 - protein, 9 aa, synthetic construct
GGTGADKFF

SEQ ID NO: 40576 - protein, 9 aa, synthetic construct
GGTGADKFI

SEQ ID NO: 40577 - protein, 9 aa, synthetic construct
GGTGADKFL

SEQ ID NO: 40578 - protein, 9 aa, synthetic construct
GGTGADKLK

SEQ ID NO: 40579 - protein, 9 aa, synthetic construct
GGTGADKMF

SEQ ID NO: 40580 - protein, 9 aa, synthetic construct
GGTGADMLW

SEQ ID NO: 40581 - protein, 9 aa, synthetic construct
GGTGADLFN

SEQ ID NO: 40582 - protein, 9 aa, synthetic construct
GGTGADLIR

SEQ ID NO: 40583 - protein, 9 aa, synthetic construct
GGTGADLLQ

SEQ ID NO: 40584 - protein, 9 aa, synthetic construct
GGTGADLMR

SEQ ID NO: 40585 - protein, 9 aa, synthetic construct
GGTGADLMV

SEQ ID NO: 40586 - protein, 9 aa, synthetic construct
GGTGADLVR

SEQ ID NO: 40587 - protein, 9 aa, synthetic construct
GGTGADLVS

SEQ ID NO: 40588 - protein, 9 aa, synthetic construct
GGTGADLYL

SEQ ID NO: 40589 - protein, 9 aa, synthetic construct
GGTGADMFG

SEQ ID NO: 40590 - protein, 9 aa, synthetic construct
GGTGADMIA

SEQ ID NO: 40591 - protein, 9 aa, synthetic construct
GGTGADMLL

SEQ ID NO: 40592 - protein, 9 aa, synthetic construct
GGTGADMLQ

SEQ ID NO: 40593 - protein, 9 aa, synthetic construct
GGTGADMLV

SEQ ID NO: 40594 - protein, 9 aa, synthetic construct
GGTGDDGVY

SEQ ID NO: 40595 - protein, 9 aa, synthetic construct
GGTGDDGYT

SEQ ID NO: 40596 - protein, 9 aa, synthetic construct
GGTGFDCAD

SEQ ID NO: 40597 - protein, 9 aa, synthetic construct
GGTGEDFLF

SEQ ID NO: 40598 - protein, 9 aa, synthetic construct
GGTGDDWMQ

SEQ ID NO: 40599 - protein, 9 aa, synthetic construct
GGTGDDWVD

SEQ ID NO: 40600 - protein, 9 aa, synthetic construct
GGTGDDWVS

SEQ ID NO: 40601 - protein, 9 aa, synthetic construct
GGTGDDYFD

SEQ ID NO: 40602 - protein, 9 aa, synthetic construct
GGTGDDYIA

SEQ ID NO: 40603 - protein, 9 aa, synthetic construct
GGTGDDYIF

SEQ ID NO: 40604 - protein, 9 aa, synthetic construct
GGTGDDYII

SEQ ID NO: 40605 - protein, 9 aa, synthetic construct
GGTGDDYIS

SEQ ID NO: 40606 - protein, 9 aa, synthetic construct
GGTGDDYIV

SEQ ID NO: 40607 - protein, 9 aa, synthetic construct
GGTGDDYLA

SEQ ID NO: 40608 - protein, 9 aa, synthetic construct
GGTGDDYLV

SEQ ID NO: 40609 - protein, 9 aa, synthetic construct
GGTGDDYMI

SEQ ID NO: 40610 - protein, 9 aa, synthetic construct
GGTGDDYML

SEQ ID NO: 40611 - protein, 9 aa, synthetic construct
GGTGDDYMN

SEQ ID NO: 40612 - protein, 9 aa, synthetic construct
GGTGDDYMQ

SEQ ID NO: 40613 - protein, 9 aa, synthetic construct
GGTGDDYVT

SEQ ID NO: 40614 - protein, 9 aa, synthetic construct
GGTGDDYYD

SEQ ID NO: 40615 - protein, 9 aa, synthetic construct
GGTGDDYYV

SEQ ID NO: 40616 - protein, 9 aa, synthetic construct
GGTGDDYYW

SEQ ID NO: 40617 - protein, 9 aa, synthetic construct
GGTGEDCLF

SEQ ID NO: 40618 - protein, 9 aa, synthetic construct
GGTGEDDLD

SEQ ID NO: 40619 - protein, 9 aa, synthetic construct
GGTGEDELA

SEQ ID NO: 40620 - protein, 9 aa, synthetic construct
GGTGEDELF

SEQ ID NO: 40621 - protein, 9 aa, synthetic construct
GGTGEDELN

SEQ ID NO: 40622 - protein, 9 aa, synthetic construct
GGTGEDELY

SEQ ID NO: 40623 - protein, 9 aa, synthetic construct
GGTGEDEMH

SEQ ID NO: 40624 - protein, 9 aa, synthetic construct
GGTGEDEVY

SEQ ID NO: 40625 - protein, 9 aa, synthetic construct
GGTGEDFID

SEQ ID NO: 40626 - protein, 9 aa, synthetic construct
GGTGEDFII

SEQ ID NO: 40627 - protein, 9 aa, synthetic construct
GGTGDDWLY

SEQ ID NO: 40628 - protein, 9 aa, synthetic construct
GGTGDDWLW

SEQ ID NO: 40629 - protein, 9 aa, synthetic construct
GGTGDDWLQ

SEQ ID NO: 40630 - protein, 9 aa, synthetic construct
GGTGDDVIQ

SEQ ID NO: 40631 - protein, 9 aa, synthetic construct
GGTGDDTFT

SEQ ID NO: 40632 - protein, 9 aa, synthetic construct
GGTGDDTIK

SEQ ID NO: 40633 - protein, 9 aa, synthetic construct
GGTGDDTIQ

SEQ ID NO: 40634 - protein, 9 aa, synthetic construct
GGTGDDTLG

SEQ ID NO: 40635 - protein, 9 aa, synthetic construct
GGTGDDTMI

SEQ ID NO: 40636 - protein, 9 aa, synthetic construct
GGTGDDTMM

SEQ ID NO: 40637 - protein, 9 aa, synthetic construct
GGTGDDTMN

SEQ ID NO: 40638 - protein, 9 aa, synthetic construct
GGTGDDTMR

SEQ ID NO: 40639 - protein, 9 aa, synthetic construct
GGTGDDTVH

SEQ ID NO: 40640 - protein, 9 aa, synthetic construct
GGTGDDTYM

SEQ ID NO: 40641 - protein, 9 aa, synthetic construct
GGTGDDVFD

SEQ ID NO: 40642 - protein, 9 aa, synthetic construct
GGTGDDVFY

SEQ ID NO: 40643 - protein, 9 aa, synthetic construct
GGTGDDVIK

SEQ ID NO: 40644 - protein, 9 aa, synthetic construct
GGTGDDVIW

SEQ ID NO: 40645 - protein, 9 aa, synthetic construct
GGTGDDWIE

SEQ ID NO: 40646 - protein, 9 aa, synthetic construct
GGTGDDVME

SEQ ID NO: 40647 - protein, 9 aa, synthetic construct
GGTGDDVMH

SEQ ID NO: 40648 - protein, 9 aa, synthetic construct
GGTGDDVMI

SEQ ID NO: 40649 - protein, 9 aa, synthetic construct
GGTGDDVMK

SEQ ID NO: 40650 - protein, 9 aa, synthetic construct
GGTGDDVML

SEQ ID NO: 40651 - protein, 9 aa, synthetic construct
GGTGDDVMN

SEQ ID NO: 40652 - protein, 9 aa, synthetic construct
GGTGDDVMQ

SEQ ID NO: 40653 - protein, 9 aa, synthetic construct
GGTGDDVMW

SEQ ID NO: 40654 - protein, 9 aa, synthetic construct
GGTGDDVVH

SEQ ID NO: 40655 - protein, 9 aa, synthetic construct
GGTGDDVVR

SEQ ID NO: 40656 - protein, 9 aa, synthetic construct
GGTGDDVVW

SEQ ID NO: 40657 - protein, 9 aa, synthetic construct
GGTGDDVVY

SEQ ID NO: 40658 - protein, 9 aa, synthetic construct
GGTGDDVYE

SEQ ID NO: 40659 - protein, 9 aa, synthetic construct
GGTGEDFIV

SEQ ID NO: 40660 - protein, 9 aa, synthetic construct
GGTGEDFMD

SEQ ID NO: 40661 - protein, 9 aa, synthetic construct
GGTGDDHFY

SEQ ID NO: 40662 - protein, 9 aa, synthetic construct
GGTGEDFVD

SEQ ID NO: 40663 - protein, 9 aa, synthetic construct
GGTGEDSLF

SEQ ID NO: 40664 - protein, 9 aa, synthetic construct
GGTGEDSLG

SEQ ID NO: 40665 - protein, 9 aa, synthetic construct
GGTGEDSLH

SEQ ID NO: 40666 - protein, 9 aa, synthetic construct
GGTGEDSLR

SEQ ID NO: 40667 - protein, 9 aa, synthetic construct
GGTGEDSLY

SEQ ID NO: 40668 - protein, 9 aa, synthetic construct
GGTGEDTFE

SEQ ID NO: 40669 - protein, 9 aa, synthetic construct
GGTGEDTFK

SEQ ID NO: 40670 - protein, 9 aa, synthetic construct
GGTGEDTII

SEQ ID NO: 40671 - protein, 9 aa, synthetic construct
GGTGEDTIL

SEQ ID NO: 40672 - protein, 9 aa, synthetic construct
GGTGEDTIS

SEQ ID NO: 40673 - protein, 9 aa, synthetic construct
GGTGEDTIT

SEQ ID NO: 40674 - protein, 9 aa, synthetic construct
GGTGEDTIW

SEQ ID NO: 40675 - protein, 9 aa, synthetic construct
GGTGEDTLR

SEQ ID NO: 40676 - protein, 9 aa, synthetic construct
GGTGEDTLV

SEQ ID NO: 40677 - protein, 9 aa, synthetic construct
GGTGEDTMD

SEQ ID NO: 40678 - protein, 9 aa, synthetic construct
GGTGEDTMV

SEQ ID NO: 40679 - protein, 9 aa, synthetic construct
GGTGEDTYI

SEQ ID NO: 40680 - protein, 9 aa, synthetic construct
GGTGEDVFR

SEQ ID NO: 40681 - protein, 9 aa, synthetic construct
GGTGEDVIF

SEQ ID NO: 40682 - protein, 9 aa, synthetic construct
GGTGEDVII

SEQ ID NO: 40683 - protein, 9 aa, synthetic construct
GGTGEDVLA

SEQ ID NO: 40684 - protein, 9 aa, synthetic construct
GGTGEDVMR

SEQ ID NO: 40685 - protein, 9 aa, synthetic construct
GGTGEDWIG

SEQ ID NO: 40686 - protein, 9 aa, synthetic construct
GGTGEDWII

SEQ ID NO: 40687 - protein, 9 aa, synthetic construct
GGTGEDWLL

SEQ ID NO: 40688 - protein, 9 aa, synthetic construct
GGTGEDWLT

SEQ ID NO: 40689 - protein, 9 aa, synthetic construct
GGTGEDYIR

SEQ ID NO: 40690 - protein, 9 aa, synthetic construct
GGTGEDYLK

SEQ ID NO: 40691 - protein, 9 aa, synthetic construct
GGTGEDYLN

SEQ ID NO: 40692 - protein, 9 aa, synthetic construct
GGTGEDSLD

SEQ ID NO: 40693 - protein, 9 aa, synthetic construct
GGTGEDRMT

SEQ ID NO: 40694 - protein, 9 aa, synthetic construct
GGTGEDRMN

SEQ ID NO: 40695 - protein, 9 aa, synthetic construct
GGTGEDLLL

SEQ ID NO: 40696 - protein, 9 aa, synthetic construct
GGTGEDGIF

SEQ ID NO: 40697 - protein, 9 aa, synthetic construct
GGTGEDGIV

SEQ ID NO: 40698 - protein, 9 aa, synthetic construct
GGTGEDGLL

SEQ ID NO: 40699 - protein, 9 aa, synthetic construct
GGTGEDHIT

SEQ ID NO: 40700 - protein, 9 aa, synthetic construct
GGTGEDHLY

SEQ ID NO: 40701 - protein, 9 aa, synthetic construct
GGTGEDIFV

SEQ ID NO: 40702 - protein, 9 aa, synthetic construct
GGTGEDIIF

SEQ ID NO: 40703 - protein, 9 aa, synthetic construct
GGTGEDIIV

SEQ ID NO: 40704 - protein, 9 aa, synthetic construct
GGTGEDILL

SEQ ID NO: 40705 - protein, 9 aa, synthetic construct
GGTGEDKID

SEQ ID NO: 40706 - protein, 9 aa, synthetic construct
GGTGEDKLW

SEQ ID NO: 40707 - protein, 9 aa, synthetic construct
GGTGEDLIF

SEQ ID NO: 40708 - protein, 9 aa, synthetic construct
GGTGEDLLF

SEQ ID NO: 40709 - protein, 9 aa, synthetic construct
GGTGEDLLT

SEQ ID NO: 40710 - protein, 9 aa, synthetic construct
GGTGEDRLQ

SEQ ID NO: 40711 - protein, 9 aa, synthetic construct
GGTGEDLLY

SEQ ID NO: 40712 - protein, 9 aa, synthetic construct
GGTGEDLML

SEQ ID NO: 40713 - protein, 9 aa, synthetic construct
GGTGEDLMQ

SEQ ID NO: 40714 - protein, 9 aa, synthetic construct
GGTGEDLMV

SEQ ID NO: 40715 - protein, 9 aa, synthetic construct
GGTGEDMAV

SEQ ID NO: 40716 - protein, 9 aa, synthetic construct
GGTGEDMLS

SEQ ID NO: 40717 - protein, 9 aa, synthetic construct
GGTGEDMLY

SEQ ID NO: 40718 - protein, 9 aa, synthetic construct
GGTGEDNLV

SEQ ID NO: 40719 - protein, 9 aa, synthetic construct
GGTGEDQIR

SEQ ID NO: 40720 - protein, 9 aa, synthetic construct
GGTGEDQVY

SEQ ID NO: 40721 - protein, 9 aa, synthetic construct
GGTGEDRFI

SEQ ID NO: 40722 - protein, 9 aa, synthetic construct
GGTGEDRIF

SEQ ID NO: 40723 - protein, 9 aa, synthetic construct
GGTGEDRLF

SEQ ID NO: 40724 - protein, 9 aa, synthetic construct
GGTGDDTFS

SEQ ID NO: 40725 - protein, 9 aa, synthetic construct
GGTGDDTFF

SEQ ID NO: 40726 - protein, 9 aa, synthetic construct
GGTGDDTFD

SEQ ID NO: 40727 - protein, 9 aa, synthetic construct
GGTGDDTFA

SEQ ID NO: 40728 - protein, 9 aa, synthetic construct
GGTGDDKYV

SEQ ID NO: 40729 - protein, 9 aa, synthetic construct
GGTGDDLAF

SEQ ID NO: 40730 - protein, 9 aa, synthetic construct
GGTGDDLAH

SEQ ID NO: 40731 - protein, 9 aa, synthetic construct
GGTGDDLAW

SEQ ID NO: 40732 - protein, 9 aa, synthetic construct
GGTGDDLFE

SEQ ID NO: 40733 - protein, 9 aa, synthetic construct
GGTGDDLFK

SEQ ID NO: 40734 - protein, 9 aa, synthetic construct
GGTGDDLFR

SEQ ID NO: 40735 - protein, 9 aa, synthetic construct
GGTGDDLFT

SEQ ID NO: 40736 - protein, 9 aa, synthetic construct
GGTGDDLIQ

SEQ ID NO: 40737 - protein, 9 aa, synthetic construct
GGTGDDLIW

SEQ ID NO: 40738 - protein, 9 aa, synthetic construct
GGTGDDLLP

SEQ ID NO: 40739 - protein, 9 aa, synthetic construct
GGTGDDLME

SEQ ID NO: 40740 - protein, 9 aa, synthetic construct
GGTGDDLMG

SEQ ID NO: 40741 - protein, 9 aa, synthetic construct
GGTGDDLMK

SEQ ID NO: 40742 - protein, 9 aa, synthetic construct
GGTGDDLMN

SEQ ID NO: 40743 - protein, 9 aa, synthetic construct
GGTGDDLMR

SEQ ID NO: 40744 - protein, 9 aa, synthetic construct
GGTGDDLMS

SEQ ID NO: 40745 - protein, 9 aa, synthetic construct
GGTGDDLVA

SEQ ID NO: 40746 - protein, 9 aa, synthetic construct
GGTGDDLVD

SEQ ID NO: 40747 - protein, 9 aa, synthetic construct
GGTGDDLVK

SEQ ID NO: 40748 - protein, 9 aa, synthetic construct
GGTGDDLVN

SEQ ID NO: 40749 - protein, 9 aa, synthetic construct
GGTGDDLVS

SEQ ID NO: 40750 - protein, 9 aa, synthetic construct
GGTGDDLYE

SEQ ID NO: 40751 - protein, 9 aa, synthetic construct
GGTGDDLYT

SEQ ID NO: 40752 - protein, 9 aa, synthetic construct
GGTGDDMAY

SEQ ID NO: 40753 - protein, 9 aa, synthetic construct
GGTGDDMFF

SEQ ID NO: 40754 - protein, 9 aa, synthetic construct
GGTGDDMFI

SEQ ID NO: 40755 - protein, 9 aa, synthetic construct
GGTGDDMID

SEQ ID NO: 40756 - protein, 9 aa, synthetic construct
GGTGDDMIL

SEQ ID NO: 40757 - protein, 9 aa, synthetic construct
GGTGDDKYF

SEQ ID NO: 40758 - protein, 9 aa, synthetic construct
GGTGDDKMY

SEQ ID NO: 40759 - protein, 9 aa, synthetic construct
GGTGDDKMW

SEQ ID NO: 40760 - protein, 9 aa, synthetic construct
GGTGDDILW

SEQ ID NO: 40761 - protein, 9 aa, synthetic construct
GGTGDDHID

SEQ ID NO: 40762 - protein, 9 aa, synthetic construct
GGTGDDHLA

SEQ ID NO: 40763 - protein, 9 aa, synthetic construct
GGTGDDHLF

SEQ ID NO: 40764 - protein, 9 aa, synthetic construct
GGTGDDHLH

SEQ ID NO: 40765 - protein, 9 aa, synthetic construct
GGTGDDHLI

SEQ ID NO: 40766 - protein, 9 aa, synthetic construct
GGTGDDHLL

SEQ ID NO: 40767 - protein, 9 aa, synthetic construct
GGTGDDHMI

SEQ ID NO: 40768 - protein, 9 aa, synthetic construct
GGTGDDHVV

SEQ ID NO: 40769 - protein, 9 aa, synthetic construct
GGTGDDIAT

SEQ ID NO: 40770 - protein, 9 aa, synthetic construct
GGTGDDIFR

SEQ ID NO: 40771 - protein, 9 aa, synthetic construct
GGTGDDIIF

SEQ ID NO: 40772 - protein, 9 aa, synthetic construct
GGTGDDIIS

SEQ ID NO: 40773 - protein, 9 aa, synthetic construct
GGTGDDILG

SEQ ID NO: 40774 - protein, 9 aa, synthetic construct
GGTGDDIMK

SEQ ID NO: 40775 - protein, 9 aa, synthetic construct
GGTGDDKMT

SEQ ID NO: 40776 - protein, 9 aa, synthetic construct
GGTGDDIVK

SEQ ID NO: 40777 - protein, 9 aa, synthetic construct
GGTGDDIVL

SEQ ID NO: 40778 - protein, 9 aa, synthetic construct
GGTGDDIVN

SEQ ID NO: 40779 - protein, 9 aa, synthetic construct
GGTGDDIVY

SEQ ID NO: 40780 - protein, 9 aa, synthetic construct
GGTGDDIYL

SEQ ID NO: 40781 - protein, 9 aa, synthetic construct
GGTGDDIYT

SEQ ID NO: 40782 - protein, 9 aa, synthetic construct
GGTGDDKFI

SEQ ID NO: 40783 - protein, 9 aa, synthetic construct
GGTGDDKIA

SEQ ID NO: 40784 - protein, 9 aa, synthetic construct
GGTGDDKIY

SEQ ID NO: 40785 - protein, 9 aa, synthetic construct
GGTGDDKLQ

SEQ ID NO: 40786 - protein, 9 aa, synthetic construct
GGTGDDKLV

SEQ ID NO: 40787 - protein, 9 aa, synthetic construct
GGTGDDKLW

SEQ ID NO: 40788 - protein, 9 aa, synthetic construct
GGTGDDKMR

SEQ ID NO: 40789 - protein, 9 aa, synthetic construct
GGTGDDMIV

SEQ ID NO: 40790 - protein, 9 aa, synthetic construct
GGTGDDMIY

SEQ ID NO: 40791 - protein, 9 aa, synthetic construct
GGTGDDMLE

SEQ ID NO: 40792 - protein, 9 aa, synthetic construct
GGTGDDSIR

SEQ ID NO: 40793 - protein, 9 aa, synthetic construct
GGTGDDRIW

SEQ ID NO: 40794 - protein, 9 aa, synthetic construct
GGTGDDRLA

SEQ ID NO: 40795 - protein, 9 aa, synthetic construct
GGTGDDRLG

SEQ ID NO: 40796 - protein, 9 aa, synthetic construct
GGTGDDRLH

SEQ ID NO: 40797 - protein, 9 aa, synthetic construct
GGTGDDRLM

SEQ ID NO: 40798 - protein, 9 aa, synthetic construct
GGTGDDRMA

SEQ ID NO: 40799 - protein, 9 aa, synthetic construct
GGTGDDRMD

SEQ ID NO: 40800 - protein, 9 aa, synthetic construct
GGTGDDRVW

SEQ ID NO: 40801 - protein, 9 aa, synthetic construct
GGTGDDRYG

SEQ ID NO: 40802 - protein, 9 aa, synthetic construct
GGTGDDRYL

SEQ ID NO: 40803 - protein, 9 aa, synthetic construct
GGTGDDSIG

SEQ ID NO: 40804 - protein, 9 aa, synthetic construct
GGTGDDSIM

SEQ ID NO: 40805 - protein, 9 aa, synthetic construct
GGTGDDSIQ

SEQ ID NO: 40806 - protein, 9 aa, synthetic construct
GGTGDDSIY

SEQ ID NO: 40807 - protein, 9 aa, synthetic construct
GGTGDDRFY

SEQ ID NO: 40808 - protein, 9 aa, synthetic construct
GGTGDDSLH

SEQ ID NO: 40809 - protein, 9 aa, synthetic construct
GGTGDDSME

SEQ ID NO: 40810 - protein, 9 aa, synthetic construct
GGTGDDSMF

SEQ ID NO: 40811 - protein, 9 aa, synthetic construct
GGTGDDSMH

SEQ ID NO: 40812 - protein, 9 aa, synthetic construct
GGTGDDSMN

SEQ ID NO: 40813 - protein, 9 aa, synthetic construct
GGTGDDSMT

SEQ ID NO: 40814 - protein, 9 aa, synthetic construct
GGTGDDSVD

SEQ ID NO: 40815 - protein, 9 aa, synthetic construct
GGTGDDSVR

SEQ ID NO: 40816 - protein, 9 aa, synthetic construct
GGTGDDSVV

SEQ ID NO: 40817 - protein, 9 aa, synthetic construct
GGTGDDSVY

SEQ ID NO: 40818 - protein, 9 aa, synthetic construct
GGTGDDSYR

SEQ ID NO: 40819 - protein, 9 aa, synthetic construct
GGTGDDSYT

SEQ ID NO: 40820 - protein, 9 aa, synthetic construct
GGTGDDTAQ

SEQ ID NO: 40821 - protein, 9 aa, synthetic construct
GGTGDDRIM

SEQ ID NO: 40822 - protein, 9 aa, synthetic construct
GGTGDDRAY

SEQ ID NO: 40823 - protein, 9 aa, synthetic construct
GGTGDDMLN

SEQ ID NO: 40824 - protein, 9 aa, synthetic construct
GGTGDDNVE

SEQ ID NO: 40825 - protein, 9 aa, synthetic construct
GGTGDDMLR

SEQ ID NO: 40826 - protein, 9 aa, synthetic construct
GGTGDDMLS

SEQ ID NO: 40827 - protein, 9 aa, synthetic construct
GGTGDDMMR

SEQ ID NO: 40828 - protein, 9 aa, synthetic construct
GGTGDDNID

SEQ ID NO: 40829 - protein, 9 aa, synthetic construct
GGTGDDNLA

SEQ ID NO: 40830 - protein, 9 aa, synthetic construct
GGTGDDNLE

SEQ ID NO: 40831 - protein, 9 aa, synthetic construct
GGTGDDNLK

SEQ ID NO: 40832 - protein, 9 aa, synthetic construct
GGTGDDNLQ

SEQ ID NO: 40833 - protein, 9 aa, synthetic construct
GGTGDDNLR

SEQ ID NO: 40834 - protein, 9 aa, synthetic construct
GGTGDDNLT

SEQ ID NO: 40835 - protein, 9 aa, synthetic construct
GGTGDDNLV

SEQ ID NO: 40836 - protein, 9 aa, synthetic construct
GGTGDDNMD

SEQ ID NO: 40837 - protein, 9 aa, synthetic construct
GGTGDDNME

SEQ ID NO: 40838 - protein, 9 aa, synthetic construct
GGTGDDNVR

SEQ ID NO: 40839 - protein, 9 aa, synthetic construct
GGTGDDRAT

SEQ ID NO: 40840 - protein, 9 aa, synthetic construct
GGTGDDPLS

SEQ ID NO: 40841 - protein, 9 aa, synthetic construct
GGTGDDQFI

SEQ ID NO: 40842 - protein, 9 aa, synthetic construct
GGTGDDQFL

SEQ ID NO: 40843 - protein, 9 aa, synthetic construct
GGTGDDQIE

SEQ ID NO: 40844 - protein, 9 aa, synthetic construct
GGTGDDQIK

SEQ ID NO: 40845 - protein, 9 aa, synthetic construct
GGTGDDQIL

SEQ ID NO: 40846 - protein, 9 aa, synthetic construct
GGTGDDQIT

SEQ ID NO: 40847 - protein, 9 aa, synthetic construct
GGTGDDQLE

SEQ ID NO: 40848 - protein, 9 aa, synthetic construct
GGTGDDQME

SEQ ID NO: 40849 - protein, 9 aa, synthetic construct
GGTGDDQMN

SEQ ID NO: 40850 - protein, 9 aa, synthetic construct
GGTGDDQMQ

SEQ ID NO: 40851 - protein, 9 aa, synthetic construct
GGTGDDQMS

SEQ ID NO: 40852 - protein, 9 aa, synthetic construct
GGTGDDRAS

SEQ ID NO: 40853 - protein, 9 aa, synthetic construct
GGTGADALR

SEQ ID NO: 40854 - protein, 9 aa, synthetic construct
GGTGADALQ

SEQ ID NO: 40855 - protein, 9 aa, synthetic construct
GGTGADALA

SEQ ID NO: 40856 - protein, 9 aa, synthetic construct
GGSGSDRFD

SEQ ID NO: 40857 - protein, 9 aa, synthetic construct
GGSGSDLLW

SEQ ID NO: 40858 - protein, 9 aa, synthetic construct
GGSGSDLVL

SEQ ID NO: 40859 - protein, 9 aa, synthetic construct
GGSGSDLYL

SEQ ID NO: 40860 - protein, 9 aa, synthetic construct
GGSGSDMFC

SEQ ID NO: 40861 - protein, 9 aa, synthetic construct
GGSGSDMFR

SEQ ID NO: 40862 - protein, 9 aa, synthetic construct
GGSGSDMIR

SEQ ID NO: 40863 - protein, 9 aa, synthetic construct
GGSGSDMIY

SEQ ID NO: 40864 - protein, 9 aa, synthetic construct
GGSGSDMLC

SEQ ID NO: 40865 - protein, 9 aa, synthetic construct
GGSGSDMLK

SEQ ID NO: 40866 - protein, 9 aa, synthetic construct
GGSGSDMLS

SEQ ID NO: 40867 - protein, 9 aa, synthetic construct
GGSGSDMLT

SEQ ID NO: 40868 - protein, 9 aa, synthetic construct
GGSGSDNAI

SEQ ID NO: 40869 - protein, 9 aa, synthetic construct
GGSGSDNAS

SEQ ID NO: 40870 - protein, 9 aa, synthetic construct
GGSGSDNFV

SEQ ID NO: 40871 - protein, 9 aa, synthetic construct
GGSGSDNLD

SEQ ID NO: 40872 - protein, 9 aa, synthetic construct
GGSGSDNLE

SEQ ID NO: 40873 - protein, 9 aa, synthetic construct
GGSGSDNLI

SEQ ID NO: 40874 - protein, 9 aa, synthetic construct
GGSGSDNLQ

SEQ ID NO: 40875 - protein, 9 aa, synthetic construct
GGSGSDNLT

SEQ ID NO: 40876 - protein, 9 aa, synthetic construct
GGSGSDNLY

SEQ ID NO: 40877 - protein, 9 aa, synthetic construct
GGSGSDQFV

SEQ ID NO: 40878 - protein, 9 aa, synthetic construct
GGSGSDQID

SEQ ID NO: 40879 - protein, 9 aa, synthetic construct
GGSGSDQIT

SEQ ID NO: 40880 - protein, 9 aa, synthetic construct
GGSGSDQLA

SEQ ID NO: 40881 - protein, 9 aa, synthetic construct
GGSGSDQLD

SEQ ID NO: 40882 - protein, 9 aa, synthetic construct
GGSGSDQLR

SEQ ID NO: 40883 - protein, 9 aa, synthetic construct
GGSGSDQLS

SEQ ID NO: 40884 - protein, 9 aa, synthetic construct
GGSGSDQMN

SEQ ID NO: 40885 - protein, 9 aa, synthetic construct
GGSGSDQMS

SEQ ID NO: 40886 - protein, 9 aa, synthetic construct
GGSGSDLIY

SEQ ID NO: 40887 - protein, 9 aa, synthetic construct
GGSGSDLIR

SEQ ID NO: 40888 - protein, 9 aa, synthetic construct
GGSGSDLID

SEQ ID NO: 40889 - protein, 9 aa, synthetic construct
GGSGSDIMV

SEQ ID NO: 40890 - protein, 9 aa, synthetic construct
GGSGSDHLQ

SEQ ID NO: 40891 - protein, 9 aa, synthetic construct
GGSGSDHLT

SEQ ID NO: 40892 - protein, 9 aa, synthetic construct
GGSGSDHLY

SEQ ID NO: 40893 - protein, 9 aa, synthetic construct
GGSGSDHVR

SEQ ID NO: 40894 - protein, 9 aa, synthetic construct
GGSGSDIAS

SEQ ID NO: 40895 - protein, 9 aa, synthetic construct
GGSGSDIFE

SEQ ID NO: 40896 - protein, 9 aa, synthetic construct
GGSGSDIFI

SEQ ID NO: 40897 - protein, 9 aa, synthetic construct
GGSGSDIIF

SEQ ID NO: 40898 - protein, 9 aa, synthetic construct
GGSGSDIIL

SEQ ID NO: 40899 - protein, 9 aa, synthetic construct
GGSGSDIIS

SEQ ID NO: 40900 - protein, 9 aa, synthetic construct
GGSGSDIIT

SEQ ID NO: 40901 - protein, 9 aa, synthetic construct
GGSGSDILK

SEQ ID NO: 40902 - protein, 9 aa, synthetic construct
GGSGSDILQ

SEQ ID NO: 40903 - protein, 9 aa, synthetic construct
GGSGSDIVD

SEQ ID NO: 40904 - protein, 9 aa, synthetic construct
GGSGSDLFI

SEQ ID NO: 40905 - protein, 9 aa, synthetic construct
GGSGSDIVE

SEQ ID NO: 40906 - protein, 9 aa, synthetic construct
GGSGSDIVI

SEQ ID NO: 40907 - protein, 9 aa, synthetic construct
GGSGSDIYL

SEQ ID NO: 40908 - protein, 9 aa, synthetic construct
GGSGSDIYN

SEQ ID NO: 40909 - protein, 9 aa, synthetic construct
GGSGSDIYR

SEQ ID NO: 40910 - protein, 9 aa, synthetic construct
GGSGSDKFV

SEQ ID NO: 40911 - protein, 9 aa, synthetic construct
GGSGSDKIG

SEQ ID NO: 40912 - protein, 9 aa, synthetic construct
GGSGSDKLD

SEQ ID NO: 40913 - protein, 9 aa, synthetic construct
GGSGSDKLE

SEQ ID NO: 40914 - protein, 9 aa, synthetic construct
GGSGSDKMI

SEQ ID NO: 40915 - protein, 9 aa, synthetic construct
GGSGSDKVK

SEQ ID NO: 40916 - protein, 9 aa, synthetic construct
GGSGSDKVY

SEQ ID NO: 40917 - protein, 9 aa, synthetic construct
GGSGSDLFA

SEQ ID NO: 40918 - protein, 9 aa, synthetic construct
GGSGSDQYT

SEQ ID NO: 40919 - protein, 9 aa, synthetic construct
GGSGSDRFF

SEQ ID NO: 40920 - protein, 9 aa, synthetic construct
GGTGADAIS

SEQ ID NO: 40921 - protein, 9 aa, synthetic construct
GGSGSDRFT

SEQ ID NO: 40922 - protein, 9 aa, synthetic construct
GGSGSDTMR

SEQ ID NO: 40923 - protein, 9 aa, synthetic construct
GGSGSDTVF

SEQ ID NO: 40924 - protein, 9 aa, synthetic construct
GGSGSDTVN

SEQ ID NO: 40925 - protein, 9 aa, synthetic construct
GGSGSDTVV

SEQ ID NO: 40926 - protein, 9 aa, synthetic construct
GGSGSDTYR

SEQ ID NO: 40927 - protein, 9 aa, synthetic construct
GGSGSDTYS

SEQ ID NO: 40928 - protein, 9 aa, synthetic construct
GGSGSDVIE

SEQ ID NO: 40929 - protein, 9 aa, synthetic construct
GGSGSDVIF

SEQ ID NO: 40930 - protein, 9 aa, synthetic construct
GGSGSDVIH

SEQ ID NO: 40931 - protein, 9 aa, synthetic construct
GGSGSDVML

SEQ ID NO: 40932 - protein, 9 aa, synthetic construct
GGSGSDVVA

SEQ ID NO: 40933 - protein, 9 aa, synthetic construct
GGSGSDVVY

SEQ ID NO: 40934 - protein, 9 aa, synthetic construct
GGSGSDVYI

SEQ ID NO: 40935 - protein, 9 aa, synthetic construct
GGSGSDWAV

SEQ ID NO: 40936 - protein, 9 aa, synthetic construct
GGSGSDWIN

SEQ ID NO: 40937 - protein, 9 aa, synthetic construct
GGSGSDWIY

SEQ ID NO: 40938 - protein, 9 aa, synthetic construct
GGSGSDWMA

SEQ ID NO: 40939 - protein, 9 aa, synthetic construct
GGSGSDYAR

SEQ ID NO: 40940 - protein, 9 aa, synthetic construct
GGSGSDYFI

SEQ ID NO: 40941 - protein, 9 aa, synthetic construct
GGSGSDYFL

SEQ ID NO: 40942 - protein, 9 aa, synthetic construct
GGSGSDYFV

SEQ ID NO: 40943 - protein, 9 aa, synthetic construct
GGSGSDYLA

SEQ ID NO: 40944 - protein, 9 aa, synthetic construct
GGSGSDYVS

SEQ ID NO: 40945 - protein, 9 aa, synthetic construct
GGSGTDAAS

SEQ ID NO: 40946 - protein, 9 aa, synthetic construct
GGSGTDALF

SEQ ID NO: 40947 - protein, 9 aa, synthetic construct
GGSGTDALH

SEQ ID NO: 40948 - protein, 9 aa, synthetic construct
GGSGTDALR

SEQ ID NO: 40949 - protein, 9 aa, synthetic construct
GGSGTDALS

SEQ ID NO: 40950 - protein, 9 aa, synthetic construct
GGSGTDDIT

SEQ ID NO: 40951 - protein, 9 aa, synthetic construct
GGSGSDTMN

SEQ ID NO: 40952 - protein, 9 aa, synthetic construct
GGSGSDTMG

SEQ ID NO: 40953 - protein, 9 aa, synthetic construct
GGSGSDTLG

SEQ ID NO: 40954 - protein, 9 aa, synthetic construct
GGSGSDSIR

SEQ ID NO: 40955 - protein, 9 aa, synthetic construct
GGSGSDRID

SEQ ID NO: 40956 - protein, 9 aa, synthetic construct
GGSGSDRIE

SEQ ID NO: 40957 - protein, 9 aa, synthetic construct
GGSGSDRIH

SEQ ID NO: 40958 - protein, 9 aa, synthetic construct
GGSGSDRIN

SEQ ID NO: 40959 - protein, 9 aa, synthetic construct
GGSGSDRIW

SEQ ID NO: 40960 - protein, 9 aa, synthetic construct
GGSGSDRLA

SEQ ID NO: 40961 - protein, 9 aa, synthetic construct
GGSGSDRLV

SEQ ID NO: 40962 - protein, 9 aa, synthetic construct
GGSGSDRLW

SEQ ID NO: 40963 - protein, 9 aa, synthetic construct
GGSGSDRMD

SEQ ID NO: 40964 - protein, 9 aa, synthetic construct
GGSGSDRMF

SEQ ID NO: 40965 - protein, 9 aa, synthetic construct
GGSGSDRVT

SEQ ID NO: 40966 - protein, 9 aa, synthetic construct
GGSGSDSFI

SEQ ID NO: 40967 - protein, 9 aa, synthetic construct
GGSGSDSIL

SEQ ID NO: 40968 - protein, 9 aa, synthetic construct
GGSGSDSIT

SEQ ID NO: 40969 - protein, 9 aa, synthetic construct
GGSGSDTIT

SEQ ID NO: 40970 - protein, 9 aa, synthetic construct
GGSGSDSIY

SEQ ID NO: 40971 - protein, 9 aa, synthetic construct
GGSGSDSLA

SEQ ID NO: 40972 - protein, 9 aa, synthetic construct
GGSGSDSMD

SEQ ID NO: 40973 - protein, 9 aa, synthetic construct
GGSGSDSMW

SEQ ID NO: 40974 - protein, 9 aa, synthetic construct
GGSGSDSVE

SEQ ID NO: 40975 - protein, 9 aa, synthetic construct
GGSGSDSVF

SEQ ID NO: 40976 - protein, 9 aa, synthetic construct
GGSGSDSVG

SEQ ID NO: 40977 - protein, 9 aa, synthetic construct
GGSGSDSVR

SEQ ID NO: 40978 - protein, 9 aa, synthetic construct
GGSGSDSYY

SEQ ID NO: 40979 - protein, 9 aa, synthetic construct
GGSGSDTFF

SEQ ID NO: 40980 - protein, 9 aa, synthetic construct
GGSGSDTFN

SEQ ID NO: 40981 - protein, 9 aa, synthetic construct
GGSGSDTIF

SEQ ID NO: 40982 - protein, 9 aa, synthetic construct
GGSGSDTII

SEQ ID NO: 40983 - protein, 9 aa, synthetic construct
GGSGSDHLN

SEQ ID NO: 40984 - protein, 9 aa, synthetic construct
GGSGSDHLI

SEQ ID NO: 40985 - protein, 9 aa, synthetic construct
GGSGSDHIE

SEQ ID NO: 40986 - protein, 9 aa, synthetic construct
GGSGSDHFV

SEQ ID NO: 40987 - protein, 9 aa, synthetic construct
GGSGRDSIE

SEQ ID NO: 40988 - protein, 9 aa, synthetic construct
GGSGRDSIF

SEQ ID NO: 40989 - protein, 9 aa, synthetic construct
GGSGRDSIG

SEQ ID NO: 40990 - protein, 9 aa, synthetic construct
GGSGRDSIR

SEQ ID NO: 40991 - protein, 9 aa, synthetic construct
GGSGRDSIS

SEQ ID NO: 40992 - protein, 9 aa, synthetic construct
GGSGRDSLD

SEQ ID NO: 40993 - protein, 9 aa, synthetic construct
GGSGRDSLH

SEQ ID NO: 40994 - protein, 9 aa, synthetic construct
GGSGRDSLQ

SEQ ID NO: 40995 - protein, 9 aa, synthetic construct
GGSGRDSLT

SEQ ID NO: 40996 - protein, 9 aa, synthetic construct
GGSGRDSMA

SEQ ID NO: 40997 - protein, 9 aa, synthetic construct
GGSGRDSMW

SEQ ID NO: 40998 - protein, 9 aa, synthetic construct
GGSGRDSVF

SEQ ID NO: 40999 - protein, 9 aa, synthetic construct
GGSGRDSVG

SEQ ID NO: 41000 - protein, 9 aa, synthetic construct
GGSGRDSVR

SEQ ID NO: 41001 - protein, 9 aa, synthetic construct
GGSGRDSVS

SEQ ID NO: 41002 - protein, 9 aa, synthetic construct
GGSGRDTAF

SEQ ID NO: 41003 - protein, 9 aa, synthetic construct
GGSGRDTAT

SEQ ID NO: 41004 - protein, 9 aa, synthetic construct
GGSGRDTFA

SEQ ID NO: 41005 - protein, 9 aa, synthetic construct
GGSGRDTFI

SEQ ID NO: 41006 - protein, 9 aa, synthetic construct
GGSGRDTFS

SEQ ID NO: 41007 - protein, 9 aa, synthetic construct
GGSGRDTFY

SEQ ID NO: 41008 - protein, 9 aa, synthetic construct
GGSGRDTIF

SEQ ID NO: 41009 - protein, 9 aa, synthetic construct
GGSGRDTIH

SEQ ID NO: 41010 - protein, 9 aa, synthetic construct
GGSGRDTIR

SEQ ID NO: 41011 - protein, 9 aa, synthetic construct
GGSGRDTIY

SEQ ID NO: 41012 - protein, 9 aa, synthetic construct
GGSGRDTLM

SEQ ID NO: 41013 - protein, 9 aa, synthetic construct
GGSGRDTMD

SEQ ID NO: 41014 - protein, 9 aa, synthetic construct
GGSGRDTMH

SEQ ID NO: 41015 - protein, 9 aa, synthetic construct
GGSGRDTVD

SEQ ID NO: 41016 - protein, 9 aa, synthetic construct
GGSGRDSFV

SEQ ID NO: 41017 - protein, 9 aa, synthetic construct
GGSGRDSAN

SEQ ID NO: 41018 - protein, 9 aa, synthetic construct
GGSGRDRYI

SEQ ID NO: 41019 - protein, 9 aa, synthetic construct
GGSGRDNVN

SEQ ID NO: 41020 - protein, 9 aa, synthetic construct
GGSGRDLLW

SEQ ID NO: 41021 - protein, 9 aa, synthetic construct
GGSGRDLMH

SEQ ID NO: 41022 - protein, 9 aa, synthetic construct
GGSGRDLMI

SEQ ID NO: 41023 - protein, 9 aa, synthetic construct
GGSGRDLMY

SEQ ID NO: 41024 - protein, 9 aa, synthetic construct
GGSGRDLVR

SEQ ID NO: 41025 - protein, 9 aa, synthetic construct
GGSGRDLYF

SEQ ID NO: 41026 - protein, 9 aa, synthetic construct
GGSGRDMIS

SEQ ID NO: 41027 - protein, 9 aa, synthetic construct
GGSGRDMLH

SEQ ID NO: 41028 - protein, 9 aa, synthetic construct
GGSGRDMLI

SEQ ID NO: 41029 - protein, 9 aa, synthetic construct
GGSGRDMLM

SEQ ID NO: 41030 - protein, 9 aa, synthetic construct
GGSGRDNIQ

SEQ ID NO: 41031 - protein, 9 aa, synthetic construct
GGSGRDNLF

SEQ ID NO: 41032 - protein, 9 aa, synthetic construct
GGSGRDNLQ

SEQ ID NO: 41033 - protein, 9 aa, synthetic construct
GGSGRDQIT

SEQ ID NO: 41034 - protein, 9 aa, synthetic construct
GGSGRDRVN

SEQ ID NO: 41035 - protein, 9 aa, synthetic construct
GGSGRDQLD

SEQ ID NO: 41036 - protein, 9 aa, synthetic construct
GGSGRDQLE

SEQ ID NO: 41037 - protein, 9 aa, synthetic construct
GGSGRDQLG

SEQ ID NO: 41038 - protein, 9 aa, synthetic construct
GGSGRDQLI

SEQ ID NO: 41039 - protein, 9 aa, synthetic construct
GGSGRDQLN

SEQ ID NO: 41040 - protein, 9 aa, synthetic construct
GGSGRDQLS

SEQ ID NO: 41041 - protein, 9 aa, synthetic construct
GGSGRDQVF

SEQ ID NO: 41042 - protein, 9 aa, synthetic construct
GGSGRDRFR

SEQ ID NO: 41043 - protein, 9 aa, synthetic construct
GGSGRDRIT

SEQ ID NO: 41044 - protein, 9 aa, synthetic construct
GGSGRDRLK

SEQ ID NO: 41045 - protein, 9 aa, synthetic construct
GGSGRDRMA

SEQ ID NO: 41046 - protein, 9 aa, synthetic construct
GGSGRDRMH

SEQ ID NO: 41047 - protein, 9 aa, synthetic construct
GGSGRDRMV

SEQ ID NO: 41048 - protein, 9 aa, synthetic construct
GGSGRDTVF

SEQ ID NO: 41049 - protein, 9 aa, synthetic construct
GGSGRDVAF

SEQ ID NO: 41050 - protein, 9 aa, synthetic construct
GGSGRDVFY

SEQ ID NO: 41051 - protein, 9 aa, synthetic construct
GGSGSDEMT

SEQ ID NO: 41052 - protein, 9 aa, synthetic construct
GGSGSDAYH

SEQ ID NO: 41053 - protein, 9 aa, synthetic construct
GGSGSDAYY

SEQ ID NO: 41054 - protein, 9 aa, synthetic construct
GGSGSDDID

SEQ ID NO: 41055 - protein, 9 aa, synthetic construct
GGSGSDDIS

SEQ ID NO: 41056 - protein, 9 aa, synthetic construct
GGSGSDDLA

SEQ ID NO: 41057 - protein, 9 aa, synthetic construct
GGSGSDDLF

SEQ ID NO: 41058 - protein, 9 aa, synthetic construct
GGSGSDDLS

SEQ ID NO: 41059 - protein, 9 aa, synthetic construct
GGSGSDEFH

SEQ ID NO: 41060 - protein, 9 aa, synthetic construct
GGSGSDEIF

SEQ ID NO: 41061 - protein, 9 aa, synthetic construct
GGSGSDEIT

SEQ ID NO: 41062 - protein, 9 aa, synthetic construct
GGSGSDEIY

SEQ ID NO: 41063 - protein, 9 aa, synthetic construct
GGSGSDELM

SEQ ID NO: 41064 - protein, 9 aa, synthetic construct
GGSGSDELS

SEQ ID NO: 41065 - protein, 9 aa, synthetic construct
GGSGSDFFD

SEQ ID NO: 41066 - protein, 9 aa, synthetic construct
GGSGSDAMT

SEQ ID NO: 41067 - protein, 9 aa, synthetic construct
GGSGSDFIA

SEQ ID NO: 41068 - protein, 9 aa, synthetic construct
GGSGSDFID

SEQ ID NO: 41069 - protein, 9 aa, synthetic construct
GGSGSDFIL

SEQ ID NO: 41070 - protein, 9 aa, synthetic construct
GGSGSDFIY

SEQ ID NO: 41071 - protein, 9 aa, synthetic construct
GGSGSDFLA

SEQ ID NO: 41072 - protein, 9 aa, synthetic construct
GGSGSDFLK

SEQ ID NO: 41073 - protein, 9 aa, synthetic construct
GGSGSDFLS

SEQ ID NO: 41074 - protein, 9 aa, synthetic construct
GGSGSDFLV

SEQ ID NO: 41075 - protein, 9 aa, synthetic construct
GGSGSDFLW

SEQ ID NO: 41076 - protein, 9 aa, synthetic construct
GGSGSDFMD

SEQ ID NO: 41077 - protein, 9 aa, synthetic construct
GGSGSDGIK

SEQ ID NO: 41078 - protein, 9 aa, synthetic construct
GGSGSDGLF

SEQ ID NO: 41079 - protein, 9 aa, synthetic construct
GGSGSDGLH

SEQ ID NO: 41080 - protein, 9 aa, synthetic construct
GGSGSDAMY

SEQ ID NO: 41081 - protein, 9 aa, synthetic construct
GGSGSDAMI

SEQ ID NO: 41082 - protein, 9 aa, synthetic construct
GGSGRDVIE

SEQ ID NO: 41083 - protein, 9 aa, synthetic construct
GGSGRDWLD

SEQ ID NO: 41084 - protein, 9 aa, synthetic construct
GGSGRDVIG

SEQ ID NO: 41085 - protein, 9 aa, synthetic construct
GGSGRDVIQ

SEQ ID NO: 41086 - protein, 9 aa, synthetic construct
GGSGRDVLF

SEQ ID NO: 41087 - protein, 9 aa, synthetic construct
GGSGRDVLI

SEQ ID NO: 41088 - protein, 9 aa, synthetic construct
GGSGRDVLK

SEQ ID NO: 41089 - protein, 9 aa, synthetic construct
GGSGRDVLR

SEQ ID NO: 41090 - protein, 9 aa, synthetic construct
GGSGRDVLW

SEQ ID NO: 41091 - protein, 9 aa, synthetic construct
GGSGRDVMI

SEQ ID NO: 41092 - protein, 9 aa, synthetic construct
GGSGRDVML

SEQ ID NO: 41093 - protein, 9 aa, synthetic construct
GGSGRDVVD

SEQ ID NO: 41094 - protein, 9 aa, synthetic construct
GGSGRDVYV

SEQ ID NO: 41095 - protein, 9 aa, synthetic construct
GGSGRDWIE

SEQ ID NO: 41096 - protein, 9 aa, synthetic construct
GGSGRDWIQ

SEQ ID NO: 41097 - protein, 9 aa, synthetic construct
GGSGRDWLN

SEQ ID NO: 41098 - protein, 9 aa, synthetic construct
GGSGSDALS

SEQ ID NO: 41099 - protein, 9 aa, synthetic construct
GGSGRDWLS

SEQ ID NO: 41100 - protein, 9 aa, synthetic construct
GGSGRDYIE

SEQ ID NO: 41101 - protein, 9 aa, synthetic construct
GGSGRDYLA

SEQ ID NO: 41102 - protein, 9 aa, synthetic construct
GGSGRDYLI

SEQ ID NO: 41103 - protein, 9 aa, synthetic construct
GGSGRDYLS

SEQ ID NO: 41104 - protein, 9 aa, synthetic construct
GGSGRDYLV

SEQ ID NO: 41105 - protein, 9 aa, synthetic construct
GGSGRDYVF

SEQ ID NO: 41106 - protein, 9 aa, synthetic construct
GGSGSDAFI

SEQ ID NO: 41107 - protein, 9 aa, synthetic construct
GGSGSDAID

SEQ ID NO: 41108 - protein, 9 aa, synthetic construct
GGSGSDAIY

SEQ ID NO: 41109 - protein, 9 aa, synthetic construct
GGSGSDALH

SEQ ID NO: 41110 - protein, 9 aa, synthetic construct
GGSGSDALN

SEQ ID NO: 41111 - protein, 9 aa, synthetic construct
GGSGSDALQ

SEQ ID NO: 41112 - protein, 9 aa, synthetic construct
GGSGTDDLK

SEQ ID NO: 41113 - protein, 9 aa, synthetic construct
GGSGTDDLV

SEQ ID NO: 41114 - protein, 9 aa, synthetic construct
GGSGTDEAA

SEQ ID NO: 41115 - protein, 9 aa, synthetic construct
GGSGVDLLD

SEQ ID NO: 41116 - protein, 9 aa, synthetic construct
GGSGVDSMT

SEQ ID NO: 41117 - protein, 9 aa, synthetic construct
GGSGVDTAE

SEQ ID NO: 41118 - protein, 9 aa, synthetic construct
GGSGVDTAN

SEQ ID NO: 41119 - protein, 9 aa, synthetic construct
GGSGVDTAY

SEQ ID NO: 41120 - protein, 9 aa, synthetic construct
GGSGVDTFH

SEQ ID NO: 41121 - protein, 9 aa, synthetic construct
GGSGVDTFI

SEQ ID NO: 41122 - protein, 9 aa, synthetic construct
GGSGVDTFV

SEQ ID NO: 41123 - protein, 9 aa, synthetic construct
GGSGVDTIV

SEQ ID NO: 41124 - protein, 9 aa, synthetic construct
GGSGVDTLE

SEQ ID NO: 41125 - protein, 9 aa, synthetic construct
GGSGVDTLF

SEQ ID NO: 41126 - protein, 9 aa, synthetic construct
GGSGVDTLL

SEQ ID NO: 41127 - protein, 9 aa, synthetic construct
GGSGVDTLN

SEQ ID NO: 41128 - protein, 9 aa, synthetic construct
GGSGVDTLQ

SEQ ID NO: 41129 - protein, 9 aa, synthetic construct
GGSGVDTLR

SEQ ID NO: 41130 - protein, 9 aa, synthetic construct
GGSGVDTLW

SEQ ID NO: 41131 - protein, 9 aa, synthetic construct
GGSGVDTMH

SEQ ID NO: 41132 - protein, 9 aa, synthetic construct
GGSGVDTMS

SEQ ID NO: 41133 - protein, 9 aa, synthetic construct
GGSGVDTMT

SEQ ID NO: 41134 - protein, 9 aa, synthetic construct
GGSGVDTVQ

SEQ ID NO: 41135 - protein, 9 aa, synthetic construct
GGSGVDTYN

SEQ ID NO: 41136 - protein, 9 aa, synthetic construct
GGSGVDVAD

SEQ ID NO: 41137 - protein, 9 aa, synthetic construct
GGSGVDVLA

SEQ ID NO: 41138 - protein, 9 aa, synthetic construct
GGSGVDVLS

SEQ ID NO: 41139 - protein, 9 aa, synthetic construct
GGSGVDVLT

SEQ ID NO: 41140 - protein, 9 aa, synthetic construct
GGSGVDVLY

SEQ ID NO: 41141 - protein, 9 aa, synthetic construct
GGSGVDVML

SEQ ID NO: 41142 - protein, 9 aa, synthetic construct
GGSGVDVVE

SEQ ID NO: 41143 - protein, 9 aa, synthetic construct
GGSGVDVVY

SEQ ID NO: 41144 - protein, 9 aa, synthetic construct
GGSGVDWLY

SEQ ID NO: 41145 - protein, 9 aa, synthetic construct
GGSGVDSLT

SEQ ID NO: 41146 - protein, 9 aa, synthetic construct
GGSGVDSLI

SEQ ID NO: 41147 - protein, 9 aa, synthetic construct
GGSGVDSIN

SEQ ID NO: 41148 - protein, 9 aa, synthetic construct
GGSGVDQIA

SEQ ID NO: 41149 - protein, 9 aa, synthetic construct
GGSGVDLLS

SEQ ID NO: 41150 - protein, 9 aa, synthetic construct
GGSGVDLLY

SEQ ID NO: 41151 - protein, 9 aa, synthetic construct
GGSGVDLMY

SEQ ID NO: 41152 - protein, 9 aa, synthetic construct
GGSGVDLVD

SEQ ID NO: 41153 - protein, 9 aa, synthetic construct
GGSGVDLVL

SEQ ID NO: 41154 - protein, 9 aa, synthetic construct
GGSGVDMLA

SEQ ID NO: 41155 - protein, 9 aa, synthetic construct
GGSGVDNII

SEQ ID NO: 41156 - protein, 9 aa, synthetic construct
GGSGVDNIQ

SEQ ID NO: 41157 - protein, 9 aa, synthetic construct
GGSGVDNLI

SEQ ID NO: 41158 - protein, 9 aa, synthetic construct
GGSGVDNLK

SEQ ID NO: 41159 - protein, 9 aa, synthetic construct
GGSGVDNLR

SEQ ID NO: 41160 - protein, 9 aa, synthetic construct
GGSGVDNLT

SEQ ID NO: 41161 - protein, 9 aa, synthetic construct
GGSGVDNMH

SEQ ID NO: 41162 - protein, 9 aa, synthetic construct
GGSGVDQLY

SEQ ID NO: 41163 - protein, 9 aa, synthetic construct
GGSGVDSIL

SEQ ID NO: 41164 - protein, 9 aa, synthetic construct
GGSGVDQMI

SEQ ID NO: 41165 - protein, 9 aa, synthetic construct
GGSGVDRAG

SEQ ID NO: 41166 - protein, 9 aa, synthetic construct
GGSGVDRFV

SEQ ID NO: 41167 - protein, 9 aa, synthetic construct
GGSGVDRIE

SEQ ID NO: 41168 - protein, 9 aa, synthetic construct
GGSGVDRIL

SEQ ID NO: 41169 - protein, 9 aa, synthetic construct
GGSGVDRIY

SEQ ID NO: 41170 - protein, 9 aa, synthetic construct
GGSGVDRLE

SEQ ID NO: 41171 - protein, 9 aa, synthetic construct
GGSGVDRLI

SEQ ID NO: 41172 - protein, 9 aa, synthetic construct
GGSGVDRLQ

SEQ ID NO: 41173 - protein, 9 aa, synthetic construct
GGSGVDRLT

SEQ ID NO: 41174 - protein, 9 aa, synthetic construct
GGSGVDRME

SEQ ID NO: 41175 - protein, 9 aa, synthetic construct
GGSGVDRMI

SEQ ID NO: 41176 - protein, 9 aa, synthetic construct
GGSGVDRVY

SEQ ID NO: 41177 - protein, 9 aa, synthetic construct
GGSGVDYIL

SEQ ID NO: 41178 - protein, 9 aa, synthetic construct
GGSGVDYLD

SEQ ID NO: 41179 - protein, 9 aa, synthetic construct
GGSGWDALY

SEQ ID NO: 41180 - protein, 9 aa, synthetic construct
GGSGYDTLH

SEQ ID NO: 41181 - protein, 9 aa, synthetic construct
GGSGYDQIL

SEQ ID NO: 41182 - protein, 9 aa, synthetic construct
GGSGYDQYD

SEQ ID NO: 41183 - protein, 9 aa, synthetic construct
GGSGYDRAH

SEQ ID NO: 41184 - protein, 9 aa, synthetic construct
GGSGYDRIY

SEQ ID NO: 41185 - protein, 9 aa, synthetic construct
GGSGYDRLD

SEQ ID NO: 41186 - protein, 9 aa, synthetic construct
GGSGYDRLN

SEQ ID NO: 41187 - protein, 9 aa, synthetic construct
GGSGYDRLY

SEQ ID NO: 41188 - protein, 9 aa, synthetic construct
GGSGYDRMY

SEQ ID NO: 41189 - protein, 9 aa, synthetic construct
GGSGYDSLA

SEQ ID NO: 41190 - protein, 9 aa, synthetic construct
GGSGYDSLD

SEQ ID NO: 41191 - protein, 9 aa, synthetic construct
GGSGYDSLI

SEQ ID NO: 41192 - protein, 9 aa, synthetic construct
GGSGYDSMY

SEQ ID NO: 41193 - protein, 9 aa, synthetic construct
GGSGYDTAE

SEQ ID NO: 41194 - protein, 9 aa, synthetic construct
GGSGYDTVG

SEQ ID NO: 41195 - protein, 9 aa, synthetic construct
GGSGYDLYW

SEQ ID NO: 41196 - protein, 9 aa, synthetic construct
GGSGYDTVR

SEQ ID NO: 41197 - protein, 9 aa, synthetic construct
GGSGYDTYI

SEQ ID NO: 41198 - protein, 9 aa, synthetic construct
GGSGYDVAY

SEQ ID NO: 41199 - protein, 9 aa, synthetic construct
GGSGYDVID

SEQ ID NO: 41200 - protein, 9 aa, synthetic construct
GGSGYDVIR

SEQ ID NO: 41201 - protein, 9 aa, synthetic construct
GGSGYDWIY

SEQ ID NO: 41202 - protein, 9 aa, synthetic construct
GGSGYDYAS

SEQ ID NO: 41203 - protein, 9 aa, synthetic construct
GGSGYDYLN

SEQ ID NO: 41204 - protein, 9 aa, synthetic construct
GGSGYDYLS

SEQ ID NO: 41205 - protein, 9 aa, synthetic construct
GGTGADAFY

SEQ ID NO: 41206 - protein, 9 aa, synthetic construct
GGTGADAID

SEQ ID NO: 41207 - protein, 9 aa, synthetic construct
GGTGADAIG

SEQ ID NO: 41208 - protein, 9 aa, synthetic construct
GGTGADAIL

SEQ ID NO: 41209 - protein, 9 aa, synthetic construct
GGSGYDNLS

SEQ ID NO: 41210 - protein, 9 aa, synthetic construct
GGSGYDLVS

SEQ ID NO: 41211 - protein, 9 aa, synthetic construct
GGSGWDEIE

SEQ ID NO: 41212 - protein, 9 aa, synthetic construct
GGSGXDFLN

SEQ ID NO: 41213 - protein, 9 aa, synthetic construct
GGSGWDKVF

SEQ ID NO: 41214 - protein, 9 aa, synthetic construct
GGSGWDMFI

SEQ ID NO: 41215 - protein, 9 aa, synthetic construct
GGSGWDNLV

SEQ ID NO: 41216 - protein, 9 aa, synthetic construct
GGSGWDNLW

SEQ ID NO: 41217 - protein, 9 aa, synthetic construct
GGSGWDQLF

SEQ ID NO: 41218 - protein, 9 aa, synthetic construct
GGSGWDSLN

SEQ ID NO: 41219 - protein, 9 aa, synthetic construct
GGSGWDTIR

SEQ ID NO: 41220 - protein, 9 aa, synthetic construct
GGSGWDTLL

SEQ ID NO: 41221 - protein, 9 aa, synthetic construct
GGSGWDTVD

SEQ ID NO: 41222 - protein, 9 aa, synthetic construct
GGSGWDVLD

SEQ ID NO: 41223 - protein, 9 aa, synthetic construct
GGSGWDVLR

SEQ ID NO: 41224 - protein, 9 aa, synthetic construct
GGSGWDVVD

SEQ ID NO: 41225 - protein, 9 aa, synthetic construct
GGSGWDWLD

SEQ ID NO: 41226 - protein, 9 aa, synthetic construct
GGSGYDAAL

SEQ ID NO: 41227 - protein, 9 aa, synthetic construct
GGSGYDLLK

SEQ ID NO: 41228 - protein, 9 aa, synthetic construct
GGSGYDAIF

SEQ ID NO: 41229 - protein, 9 aa, synthetic construct
GGSGYDDLD

SEQ ID NO: 41230 - protein, 9 aa, synthetic construct
GGSGYDDLS

SEQ ID NO: 41231 - protein, 9 aa, synthetic construct
GGSGYDELH

SEQ ID NO: 41232 - protein, 9 aa, synthetic construct
GGSGYDELR

SEQ ID NO: 41233 - protein, 9 aa, synthetic construct
GGSGYDEMY

SEQ ID NO: 41234 - protein, 9 aa, synthetic construct
GGSGYDGLD

SEQ ID NO: 41235 - protein, 9 aa, synthetic construct
GGSGYDILN

SEQ ID NO: 41236 - protein, 9 aa, synthetic construct
GGSGYDILS

SEQ ID NO: 41237 - protein, 9 aa, synthetic construct
GGSGYDIVD

SEQ ID NO: 41238 - protein, 9 aa, synthetic construct
GGSGYDKIF

SEQ ID NO: 41239 - protein, 9 aa, synthetic construct
GGSGYDKLT

SEQ ID NO: 41240 - protein, 9 aa, synthetic construct
GGSGYDKLY

SEQ ID NO: 41241 - protein, 9 aa, synthetic construct
GGSGVDLLR

SEQ ID NO: 41242 - protein, 9 aa, synthetic construct
GGSGVDLLA

SEQ ID NO: 41243 - protein, 9 aa, synthetic construct
GGSGTDELD

SEQ ID NO: 41244 - protein, 9 aa, synthetic construct
GGSGVDLID

SEQ ID NO: 41245 - protein, 9 aa, synthetic construct
GGSGTDLLF

SEQ ID NO: 41246 - protein, 9 aa, synthetic construct
GGSGTDLLM

SEQ ID NO: 41247 - protein, 9 aa, synthetic construct
GGSGTDLLY

SEQ ID NO: 41248 - protein, 9 aa, synthetic construct
GGSGTDLVD

SEQ ID NO: 41249 - protein, 9 aa, synthetic construct
GGSGTDMLY

SEQ ID NO: 41250 - protein, 9 aa, synthetic construct
GGSGTDNII

SEQ ID NO: 41251 - protein, 9 aa, synthetic construct
GGSGTDNLI

SEQ ID NO: 41252 - protein, 9 aa, synthetic construct
GGSGTDNLS

SEQ ID NO: 41253 - protein, 9 aa, synthetic construct
GGSGTDNLY

SEQ ID NO: 41254 - protein, 9 aa, synthetic construct
GGSGTDQLF

SEQ ID NO: 41255 - protein, 9 aa, synthetic construct
GGSGTDQLS

SEQ ID NO: 41256 - protein, 9 aa, synthetic construct
GGSGTDQLT

SEQ ID NO: 41257 - protein, 9 aa, synthetic construct
GGSGTDQMC

SEQ ID NO: 41258 - protein, 9 aa, synthetic construct
GGSGTDRFY

SEQ ID NO: 41259 - protein, 9 aa, synthetic construct
GGSGTDRIS

SEQ ID NO: 41260 - protein, 9 aa, synthetic construct
GGSGTDRLL

SEQ ID NO: 41261 - protein, 9 aa, synthetic construct
GGSGTDRMM

SEQ ID NO: 41262 - protein, 9 aa, synthetic construct
GGSGTDRVT

SEQ ID NO: 41263 - protein, 9 aa, synthetic construct
GGSGTDSIR

SEQ ID NO: 41264 - protein, 9 aa, synthetic construct
GGSGTDSIY

SEQ ID NO: 41265 - protein, 9 aa, synthetic construct
GGSGTDSLL

SEQ ID NO: 41266 - protein, 9 aa, synthetic construct
GGSGTDTAE

SEQ ID NO: 41267 - protein, 9 aa, synthetic construct
GGSGTDTAF

SEQ ID NO: 41268 - protein, 9 aa, synthetic construct
GGSGTDTAQ

SEQ ID NO: 41269 - protein, 9 aa, synthetic construct
GGSGTDTAY

SEQ ID NO: 41270 - protein, 9 aa, synthetic construct
GGSGTDTFH

SEQ ID NO: 41271 - protein, 9 aa, synthetic construct
GGSGTDTFK

SEQ ID NO: 41272 - protein, 9 aa, synthetic construct
GGSGTDTIA

SEQ ID NO: 41273 - protein, 9 aa, synthetic construct
GGSGTDTIF

SEQ ID NO: 41274 - protein, 9 aa, synthetic construct
GGSGTDLLE

SEQ ID NO: 41275 - protein, 9 aa, synthetic construct
GGSGTDLLA

SEQ ID NO: 41276 - protein, 9 aa, synthetic construct
GGSGTDLFR

SEQ ID NO: 41277 - protein, 9 aa, synthetic construct
GGSGTDIAF

SEQ ID NO: 41278 - protein, 9 aa, synthetic construct
GGSGTDELF

SEQ ID NO: 41279 - protein, 9 aa, synthetic construct
GGSGTDELH

SEQ ID NO: 41280 - protein, 9 aa, synthetic construct
GGSGTDELN

SEQ ID NO: 41281 - protein, 9 aa, synthetic construct
GGSGTDELR

SEQ ID NO: 41282 - protein, 9 aa, synthetic construct
GGSGTDELT

SEQ ID NO: 41283 - protein, 9 aa, synthetic construct
GGSGTDFIF

SEQ ID NO: 41284 - protein, 9 aa, synthetic construct
GGSGTDFIS

SEQ ID NO: 41285 - protein, 9 aa, synthetic construct
GGSGTDFMF

SEQ ID NO: 41286 - protein, 9 aa, synthetic construct
GGSGTDGLG

SEQ ID NO: 41287 - protein, 9 aa, synthetic construct
GGSGTDHLI

SEQ ID NO: 41288 - protein, 9 aa, synthetic construct
GGSGTDHLL

SEQ ID NO: 41289 - protein, 9 aa, synthetic construct
GGSGTDHLV

SEQ ID NO: 41290 - protein, 9 aa, synthetic construct
GGSGTDHMT

SEQ ID NO: 41291 - protein, 9 aa, synthetic construct
GGSGTDIAK

SEQ ID NO: 41292 - protein, 9 aa, synthetic construct
GGSGTDKVY

SEQ ID NO: 41293 - protein, 9 aa, synthetic construct
GGSGTDIAS

SEQ ID NO: 41294 - protein, 9 aa, synthetic construct
GGSGTDIID

SEQ ID NO: 41295 - protein, 9 aa, synthetic construct
GGSGTDIIF

SEQ ID NO: 41296 - protein, 9 aa, synthetic construct
GGSGTDILA

SEQ ID NO: 41297 - protein, 9 aa, synthetic construct
GGSGTDILL

SEQ ID NO: 41298 - protein, 9 aa, synthetic construct
GGSGTDILS

SEQ ID NO: 41299 - protein, 9 aa, synthetic construct
GGSGTDILT

SEQ ID NO: 41300 - protein, 9 aa, synthetic construct
GGSGTDIMQ

SEQ ID NO: 41301 - protein, 9 aa, synthetic construct
GGSGTDIVF

SEQ ID NO: 41302 - protein, 9 aa, synthetic construct
GGSGTDIVH

SEQ ID NO: 41303 - protein, 9 aa, synthetic construct
GGSGTDIVS

SEQ ID NO: 41304 - protein, 9 aa, synthetic construct
GGSGTDKIK

SEQ ID NO: 41305 - protein, 9 aa, synthetic construct
GGSGTDKLF

SEQ ID NO: 41306 - protein, 9 aa, synthetic construct
GGSGTDTIL

SEQ ID NO: 41307 - protein, 9 aa, synthetic construct
GGSGTDTIY

SEQ ID NO: 41308 - protein, 9 aa, synthetic construct
GGSGTDTLF

SEQ ID NO: 41309 - protein, 9 aa, synthetic construct
GGSGVDHIY

SEQ ID NO: 41310 - protein, 9 aa, synthetic construct
GGSGVDEII

SEQ ID NO: 41311 - protein, 9 aa, synthetic construct
GGSGVDELN

SEQ ID NO: 41312 - protein, 9 aa, synthetic construct
GGSGVDELY

SEQ ID NO: 41313 - protein, 9 aa, synthetic construct
GGSGVDEMA

SEQ ID NO: 41314 - protein, 9 aa, synthetic construct
GGSGVDEMR

SEQ ID NO: 41315 - protein, 9 aa, synthetic construct
GGSGVDEVI

SEQ ID NO: 41316 - protein, 9 aa, synthetic construct
GGSGVDFAD

SEQ ID NO: 41317 - protein, 9 aa, synthetic construct
GGSGVDFAV

SEQ ID NO: 41318 - protein, 9 aa, synthetic construct
GGSGVDFLI

SEQ ID NO: 41319 - protein, 9 aa, synthetic construct
GGSGVDFLQ

SEQ ID NO: 41320 - protein, 9 aa, synthetic construct
GGSGVDFVL

SEQ ID NO: 41321 - protein, 9 aa, synthetic construct
GGSGVDGLT

SEQ ID NO: 41322 - protein, 9 aa, synthetic construct
GGSGVDGLV

SEQ ID NO: 41323 - protein, 9 aa, synthetic construct
GGSGVDHLI

SEQ ID NO: 41324 - protein, 9 aa, synthetic construct
GGSGVDDLH

SEQ ID NO: 41325 - protein, 9 aa, synthetic construct
GGSGVDHLS

SEQ ID NO: 41326 - protein, 9 aa, synthetic construct
GGSGVDHLY

SEQ ID NO: 41327 - protein, 9 aa, synthetic construct
GGSGVDIAR

SEQ ID NO: 41328 - protein, 9 aa, synthetic construct
GGSGVDIAS

SEQ ID NO: 41329 - protein, 9 aa, synthetic construct
GGSGVDILI

SEQ ID NO: 41330 - protein, 9 aa, synthetic construct
GGSGVDILK

SEQ ID NO: 41331 - protein, 9 aa, synthetic construct
GGSGVDILN

SEQ ID NO: 41332 - protein, 9 aa, synthetic construct
GGSGVDIMD

SEQ ID NO: 41333 - protein, 9 aa, synthetic construct
GGSGVDKLN

SEQ ID NO: 41334 - protein, 9 aa, synthetic construct
GGSGVDKLS

SEQ ID NO: 41335 - protein, 9 aa, synthetic construct
GGSGVDLAF

SEQ ID NO: 41336 - protein, 9 aa, synthetic construct
GGSGVDLFE

SEQ ID NO: 41337 - protein, 9 aa, synthetic construct
GGSGVDLFL

SEQ ID NO: 41338 - protein, 9 aa, synthetic construct
GGSGVDDLT

SEQ ID NO: 41339 - protein, 9 aa, synthetic construct
GGSGVDDIT

SEQ ID NO: 41340 - protein, 9 aa, synthetic construct
GGSGTDTMD

SEQ ID NO: 41341 - protein, 9 aa, synthetic construct
GGSGTDVVG

SEQ ID NO: 41342 - protein, 9 aa, synthetic construct
GGSGTDTMR

SEQ ID NO: 41343 - protein, 9 aa, synthetic construct
GGSGTDTMY

SEQ ID NO: 41344 - protein, 9 aa, synthetic construct
GGSGTDTYT

SEQ ID NO: 41345 - protein, 9 aa, synthetic construct
GGSGTDTYV

SEQ ID NO: 41346 - protein, 9 aa, synthetic construct
GGSGTDVAF

SEQ ID NO: 41347 - protein, 9 aa, synthetic construct
GGSGTDVAI

SEQ ID NO: 41348 - protein, 9 aa, synthetic construct
GGSGTDVFM

SEQ ID NO: 41349 - protein, 9 aa, synthetic construct
GGSGTDVFS

SEQ ID NO: 41350 - protein, 9 aa, synthetic construct
GGSGTDVIA

SEQ ID NO: 41351 - protein, 9 aa, synthetic construct
GGSGTDVIY

SEQ ID NO: 41352 - protein, 9 aa, synthetic construct
GGSGTDVLF

SEQ ID NO: 41353 - protein, 9 aa, synthetic construct
GGSGTDVLT

SEQ ID NO: 41354 - protein, 9 aa, synthetic construct
GGSGTDVVA

SEQ ID NO: 41355 - protein, 9 aa, synthetic construct
GGSGTDVVI

SEQ ID NO: 41356 - protein, 9 aa, synthetic construct
GGSGVDAVS

SEQ ID NO: 41357 - protein, 9 aa, synthetic construct
GGSGTDWAN

SEQ ID NO: 41358 - protein, 9 aa, synthetic construct
GGSGTDWLL

SEQ ID NO: 41359 - protein, 9 aa, synthetic construct
GGSGTDWLS

SEQ ID NO: 41360 - protein, 9 aa, synthetic construct
GGSGTDWVS

SEQ ID NO: 41361 - protein, 9 aa, synthetic construct
GGSGTDWVY

SEQ ID NO: 41362 - protein, 9 aa, synthetic construct
GGSGTDYAV

SEQ ID NO: 41363 - protein, 9 aa, synthetic construct
GGSGTDYLK

SEQ ID NO: 41364 - protein, 9 aa, synthetic construct
GGSGTDYLL

SEQ ID NO: 41365 - protein, 9 aa, synthetic construct
GGSGTDYVR

SEQ ID NO: 41366 - protein, 9 aa, synthetic construct
GGSGVDAIS

SEQ ID NO: 41367 - protein, 9 aa, synthetic construct
GGSGVDALS

SEQ ID NO: 41368 - protein, 9 aa, synthetic construct
GGSGVDALT

SEQ ID NO: 41369 - protein, 9 aa, synthetic construct
GGSGVDAMA

SEQ ID NO: 41370 - protein, 9 aa, synthetic construct
GGTGFDAID

SEQ ID NO: 41371 - protein, 9 aa, synthetic construct
GGTGFDELH

SEQ ID NO: 41372 - protein, 9 aa, synthetic construct
GGTGSDIYI

SEQ ID NO: 41373 - protein, 9 aa, synthetic construct
GGTGNDVIL

SEQ ID NO: 41374 - protein, 9 aa, synthetic construct
GGTGNDSYE

SEQ ID NO: 41375 - protein, 9 aa, synthetic construct
GGTGNDTAF

SEQ ID NO: 41376 - protein, 9 aa, synthetic construct
GGTGNDTAL

SEQ ID NO: 41377 - protein, 9 aa, synthetic construct
GGTGNDTAV

SEQ ID NO: 41378 - protein, 9 aa, synthetic construct
GGTGNDTFD

SEQ ID NO: 41379 - protein, 9 aa, synthetic construct
GGTGNDTFG

SEQ ID NO: 41380 - protein, 9 aa, synthetic construct
GGTGNDTFK

SEQ ID NO: 41381 - protein, 9 aa, synthetic construct
GGTGNDTFM

SEQ ID NO: 41382 - protein, 9 aa, synthetic construct
GGTGNDTFN

SEQ ID NO: 41383 - protein, 9 aa, synthetic construct
GGTGNDTFW

SEQ ID NO: 41384 - protein, 9 aa, synthetic construct
GGTGNDTIM

SEQ ID NO: 41385 - protein, 9 aa, synthetic construct
GGTGNDTLC

SEQ ID NO: 41386 - protein, 9 aa, synthetic construct
GGTGNDTMG

SEQ ID NO: 41387 - protein, 9 aa, synthetic construct
GGTGNDTMH

SEQ ID NO: 41388 - protein, 9 aa, synthetic construct
GGTGNDTMW

SEQ ID NO: 41389 - protein, 9 aa, synthetic construct
GGTGNDTVM

SEQ ID NO: 41390 - protein, 9 aa, synthetic construct
GGTGNDTVV

SEQ ID NO: 41391 - protein, 9 aa, synthetic construct
GGTGNDTYE

SEQ ID NO: 41392 - protein, 9 aa, synthetic construct
GGTGNDVAD

SEQ ID NO: 41393 - protein, 9 aa, synthetic construct
GGTGNDVAE

SEQ ID NO: 41394 - protein, 9 aa, synthetic construct
GGTGNDVAK

SEQ ID NO: 41395 - protein, 9 aa, synthetic construct
GGTGNDVAN

SEQ ID NO: 41396 - protein, 9 aa, synthetic construct
GGTGNDVAT

SEQ ID NO: 41397 - protein, 9 aa, synthetic construct
GGTGNDVFD

SEQ ID NO: 41398 - protein, 9 aa, synthetic construct
GGTGNDVFQ

SEQ ID NO: 41399 - protein, 9 aa, synthetic construct
GGTGNDVFW

SEQ ID NO: 41400 - protein, 9 aa, synthetic construct
GGTGNDVIA

SEQ ID NO: 41401 - protein, 9 aa, synthetic construct
GGTGNDVIF

SEQ ID NO: 41402 - protein, 9 aa, synthetic construct
GGTGNDVIG

SEQ ID NO: 41403 - protein, 9 aa, synthetic construct
GGTGNDSVY

SEQ ID NO: 41404 - protein, 9 aa, synthetic construct
GGTGNDSVW

SEQ ID NO: 41405 - protein, 9 aa, synthetic construct
GGTGNDSVV

SEQ ID NO: 41406 - protein, 9 aa, synthetic construct
GGTGNDSAH

SEQ ID NO: 41407 - protein, 9 aa, synthetic construct
GGTGNDRIG

SEQ ID NO: 41408 - protein, 9 aa, synthetic construct
GGTGNDRIL

SEQ ID NO: 41409 - protein, 9 aa, synthetic construct
GGTGNDRIW

SEQ ID NO: 41410 - protein, 9 aa, synthetic construct
GGTGNDRMK

SEQ ID NO: 41411 - protein, 9 aa, synthetic construct
GGTGNDRMR

SEQ ID NO: 41412 - protein, 9 aa, synthetic construct
GGTGNDRMW

SEQ ID NO: 41413 - protein, 9 aa, synthetic construct
GGTGNDRVD

SEQ ID NO: 41414 - protein, 9 aa, synthetic construct
GGTGNDRVE

SEQ ID NO: 41415 - protein, 9 aa, synthetic construct
GGTGNDRVI

SEQ ID NO: 41416 - protein, 9 aa, synthetic construct
GGTGNDRVR

SEQ ID NO: 41417 - protein, 9 aa, synthetic construct
GGTGNDRVT

SEQ ID NO: 41418 - protein, 9 aa, synthetic construct
GGTGNDRYE

SEQ ID NO: 41419 - protein, 9 aa, synthetic construct
GGTGNDRYY

SEQ ID NO: 41420 - protein, 9 aa, synthetic construct
GGTGNDSFY

SEQ ID NO: 41421 - protein, 9 aa, synthetic construct
GGTGNDSVQ

SEQ ID NO: 41422 - protein, 9 aa, synthetic construct
GGTGNDSIG

SEQ ID NO: 41423 - protein, 9 aa, synthetic construct
GGTGNDSIW

SEQ ID NO: 41424 - protein, 9 aa, synthetic construct
GGTGNDSLH

SEQ ID NO: 41425 - protein, 9 aa, synthetic construct
GGTGNDSME

SEQ ID NO: 41426 - protein, 9 aa, synthetic construct
GGTGNDSMH

SEQ ID NO: 41427 - protein, 9 aa, synthetic construct
GGTGNDSMR

SEQ ID NO: 41428 - protein, 9 aa, synthetic construct
GGTGNDSVA

SEQ ID NO: 41429 - protein, 9 aa, synthetic construct
GGTGNDSVD

SEQ ID NO: 41430 - protein, 9 aa, synthetic construct
GGTGNDSVE

SEQ ID NO: 41431 - protein, 9 aa, synthetic construct
GGTGNDSVF

SEQ ID NO: 41432 - protein, 9 aa, synthetic construct
GGTGNDSVG

SEQ ID NO: 41433 - protein, 9 aa, synthetic construct
GGTGNDSVI

SEQ ID NO: 41434 - protein, 9 aa, synthetic construct
GGTGNDSVM

SEQ ID NO: 41435 - protein, 9 aa, synthetic construct
GGTGNDVII

SEQ ID NO: 41436 - protein, 9 aa, synthetic construct
GGTGNDVMF

SEQ ID NO: 41437 - protein, 9 aa, synthetic construct
GGTGQDELH

SEQ ID NO: 41438 - protein, 9 aa, synthetic construct
GGTGNDVMG

SEQ ID NO: 41439 - protein, 9 aa, synthetic construct
GGTGNDYVH

SEQ ID NO: 41440 - protein, 9 aa, synthetic construct
GGTGNDYVL

SEQ ID NO: 41441 - protein, 9 aa, synthetic construct
GGTGNDYYM

SEQ ID NO: 41442 - protein, 9 aa, synthetic construct
GGTGNDYYV

SEQ ID NO: 41443 - protein, 9 aa, synthetic construct
GGTGPDALT

SEQ ID NO: 41444 - protein, 9 aa, synthetic construct
GGTGPDAMV

SEQ ID NO: 41445 - protein, 9 aa, synthetic construct
GGTGPDDLD

SEQ ID NO: 41446 - protein, 9 aa, synthetic construct
GGTGPDHIR

SEQ ID NO: 41447 - protein, 9 aa, synthetic construct
GGTGPDIFL

SEQ ID NO: 41448 - protein, 9 aa, synthetic construct
GGTGPDLLT

SEQ ID NO: 41449 - protein, 9 aa, synthetic construct
GGTGPDLLV

SEQ ID NO: 41450 - protein, 9 aa, synthetic construct
GGTGPDNMI

SEQ ID NO: 41451 - protein, 9 aa, synthetic construct
GGTGPDRFD

SEQ ID NO: 41452 - protein, 9 aa, synthetic construct
GGTGPDSLS

SEQ ID NO: 41453 - protein, 9 aa, synthetic construct
GGTGPDSLV

SEQ ID NO: 41454 - protein, 9 aa, synthetic construct
GGTGPDTFG

SEQ ID NO: 41455 - protein, 9 aa, synthetic construct
GGTGPDTLA

SEQ ID NO: 41456 - protein, 9 aa, synthetic construct
GGTGPDTLI

SEQ ID NO: 41457 - protein, 9 aa, synthetic construct
GGTGPDTLK

SEQ ID NO: 41458 - protein, 9 aa, synthetic construct
GGTGPDTLL

SEQ ID NO: 41459 - protein, 9 aa, synthetic construct
GGTGPDTLN

SEQ ID NO: 41460 - protein, 9 aa, synthetic construct
GGTGPDTLS

SEQ ID NO: 41461 - protein, 9 aa, synthetic construct
GGTGPDVFV

SEQ ID NO: 41462 - protein, 9 aa, synthetic construct
GGTGQDALF

SEQ ID NO: 41463 - protein, 9 aa, synthetic construct
GGTGQDALT

SEQ ID NO: 41464 - protein, 9 aa, synthetic construct
GGTGQDAMR

SEQ ID NO: 41465 - protein, 9 aa, synthetic construct
GGTGQDDIY

SEQ ID NO: 41466 - protein, 9 aa, synthetic construct
GGTGQDDLS

SEQ ID NO: 41467 - protein, 9 aa, synthetic construct
GGTGQDDMH

SEQ ID NO: 41468 - protein, 9 aa, synthetic construct
GGTGNDYVF

SEQ ID NO: 41469 - protein, 9 aa, synthetic construct
GGTGNDYML

SEQ ID NO: 41470 - protein, 9 aa, synthetic construct
GGTGNDYIV

SEQ ID NO: 41471 - protein, 9 aa, synthetic construct
GGTGNDWIN

SEQ ID NO: 41472 - protein, 9 aa, synthetic construct
GGTGNDVMY

SEQ ID NO: 41473 - protein, 9 aa, synthetic construct
GGTGNDVVD

SEQ ID NO: 41474 - protein, 9 aa, synthetic construct
GGTGNDVVF

SEQ ID NO: 41475 - protein, 9 aa, synthetic construct
GGTGNDVVR

SEQ ID NO: 41476 - protein, 9 aa, synthetic construct
GGTGNDVVV

SEQ ID NO: 41477 - protein, 9 aa, synthetic construct
GGTGNDVYA

SEQ ID NO: 41478 - protein, 9 aa, synthetic construct
GGTGNDVYK

SEQ ID NO: 41479 - protein, 9 aa, synthetic construct
GGTGNDVYQ

SEQ ID NO: 41480 - protein, 9 aa, synthetic construct
GGTGNDVYT

SEQ ID NO: 41481 - protein, 9 aa, synthetic construct
GGTGNDWAL

SEQ ID NO: 41482 - protein, 9 aa, synthetic construct
GGTGNDWAV

SEQ ID NO: 41483 - protein, 9 aa, synthetic construct
GGTGNDWFY

SEQ ID NO: 41484 - protein, 9 aa, synthetic construct
GGTGNDWIA

SEQ ID NO: 41485 - protein, 9 aa, synthetic construct
GGTGNDWIR

SEQ ID NO: 41486 - protein, 9 aa, synthetic construct
GGTGNDYIT

SEQ ID NO: 41487 - protein, 9 aa, synthetic construct
GGTGNDWLI

SEQ ID NO: 41488 - protein, 9 aa, synthetic construct
GGTGNDWLT

SEQ ID NO: 41489 - protein, 9 aa, synthetic construct
GGTGNDWLV

SEQ ID NO: 41490 - protein, 9 aa, synthetic construct
GGTGNDWMS

SEQ ID NO: 41491 - protein, 9 aa, synthetic construct
GGTGNDWMT

SEQ ID NO: 41492 - protein, 9 aa, synthetic construct
GGTGNDWMV

SEQ ID NO: 41493 - protein, 9 aa, synthetic construct
GGTGNDWVG

SEQ ID NO: 41494 - protein, 9 aa, synthetic construct
GGTGNDWYF

SEQ ID NO: 41495 - protein, 9 aa, synthetic construct
GGTGNDYAL

SEQ ID NO: 41496 - protein, 9 aa, synthetic construct
GGTGNDYFD

SEQ ID NO: 41497 - protein, 9 aa, synthetic construct
GGTGNDYFV

SEQ ID NO: 41498 - protein, 9 aa, synthetic construct
GGTGNDYIK

SEQ ID NO: 41499 - protein, 9 aa, synthetic construct
GGTGNDYIR

SEQ ID NO: 41500 - protein, 9 aa, synthetic construct
GGTGNDRIA

SEQ ID NO: 41501 - protein, 9 aa, synthetic construct
GGTGNDRFY

SEQ ID NO: 41502 - protein, 9 aa, synthetic construct
GGTGNDRFS

SEQ ID NO: 41503 - protein, 9 aa, synthetic construct
GGTGNDRFD

SEQ ID NO: 41504 - protein, 9 aa, synthetic construct
GGTGNDHMI

SEQ ID NO: 41505 - protein, 9 aa, synthetic construct
GGTGNDHMS

SEQ ID NO: 41506 - protein, 9 aa, synthetic construct
GGTGNDHYD

SEQ ID NO: 41507 - protein, 9 aa, synthetic construct
GGTGNDHYY

SEQ ID NO: 41508 - protein, 9 aa, synthetic construct
GGTGNDIAF

SEQ ID NO: 41509 - protein, 9 aa, synthetic construct
GGTGNDIAI

SEQ ID NO: 41510 - protein, 9 aa, synthetic construct
GGTGNDIAL

SEQ ID NO: 41511 - protein, 9 aa, synthetic construct
GGTGNDIAY

SEQ ID NO: 41512 - protein, 9 aa, synthetic construct
GGTGNDIFA

SEQ ID NO: 41513 - protein, 9 aa, synthetic construct
GGTGNDIFD

SEQ ID NO: 41514 - protein, 9 aa, synthetic construct
GGTGNDIFL

SEQ ID NO: 41515 - protein, 9 aa, synthetic construct
GGTGNDIIA

SEQ ID NO: 41516 - protein, 9 aa, synthetic construct
GGTGNDIIH

SEQ ID NO: 41517 - protein, 9 aa, synthetic construct
GGTGNDIIQ

SEQ ID NO: 41518 - protein, 9 aa, synthetic construct
GGTGNDILG

SEQ ID NO: 41519 - protein, 9 aa, synthetic construct
GGTGNDIMA

SEQ ID NO: 41520 - protein, 9 aa, synthetic construct
GGTGNDIMD

SEQ ID NO: 41521 - protein, 9 aa, synthetic construct
GGTGNDIMH

SEQ ID NO: 41522 - protein, 9 aa, synthetic construct
GGTGNDIMN

SEQ ID NO: 41523 - protein, 9 aa, synthetic construct
GGTGNDIVC

SEQ ID NO: 41524 - protein, 9 aa, synthetic construct
GGTGNDIYL

SEQ ID NO: 41525 - protein, 9 aa, synthetic construct
GGTGNDIYQ

SEQ ID NO: 41526 - protein, 9 aa, synthetic construct
GGTGNDIYR

SEQ ID NO: 41527 - protein, 9 aa, synthetic construct
GGTGNDKIE

SEQ ID NO: 41528 - protein, 9 aa, synthetic construct
GGTGNDKIS

SEQ ID NO: 41529 - protein, 9 aa, synthetic construct
GGTGNDKIT

SEQ ID NO: 41530 - protein, 9 aa, synthetic construct
GGTGNDKIV

SEQ ID NO: 41531 - protein, 9 aa, synthetic construct
GGTGNDKLE

SEQ ID NO: 41532 - protein, 9 aa, synthetic construct
GGTGNDKLI

SEQ ID NO: 41533 - protein, 9 aa, synthetic construct
GGTGNDHMA

SEQ ID NO: 41534 - protein, 9 aa, synthetic construct
GGTGNDHLR

SEQ ID NO: 41535 - protein, 9 aa, synthetic construct
GGTGNDHLQ

SEQ ID NO: 41536 - protein, 9 aa, synthetic construct
GGTGNDFVD

SEQ ID NO: 41537 - protein, 9 aa, synthetic construct
GGTGNDFAR

SEQ ID NO: 41538 - protein, 9 aa, synthetic construct
GGTGNDFAS

SEQ ID NO: 41539 - protein, 9 aa, synthetic construct
GGTGNDFAY

SEQ ID NO: 41540 - protein, 9 aa, synthetic construct
GGTGNDFII

SEQ ID NO: 41541 - protein, 9 aa, synthetic construct
GGTGNDFIM

SEQ ID NO: 41542 - protein, 9 aa, synthetic construct
GGTGNDFIW

SEQ ID NO: 41543 - protein, 9 aa, synthetic construct
GGTGNDFIY

SEQ ID NO: 41544 - protein, 9 aa, synthetic construct
GGTGNDFLL

SEQ ID NO: 41545 - protein, 9 aa, synthetic construct
GGTGNDFMN

SEQ ID NO: 41546 - protein, 9 aa, synthetic construct
GGTGNDFMR

SEQ ID NO: 41547 - protein, 9 aa, synthetic construct
GGTGNDFMS

SEQ ID NO: 41548 - protein, 9 aa, synthetic construct
GGTGNDFMT

SEQ ID NO: 41549 - protein, 9 aa, synthetic construct
GGTGNDFMV

SEQ ID NO: 41550 - protein, 9 aa, synthetic construct
GGTGNDFVF

SEQ ID NO: 41551 - protein, 9 aa, synthetic construct
GGTGNDHLM

SEQ ID NO: 41552 - protein, 9 aa, synthetic construct
GGTGNDFVS

SEQ ID NO: 41553 - protein, 9 aa, synthetic construct
GGTGNDFYF

SEQ ID NO: 41554 - protein, 9 aa, synthetic construct
GGTGNDFYT

SEQ ID NO: 41555 - protein, 9 aa, synthetic construct
GGTGNDFYY

SEQ ID NO: 41556 - protein, 9 aa, synthetic construct
GGTGNDGLR

SEQ ID NO: 41557 - protein, 9 aa, synthetic construct
GGTGNDGVF

SEQ ID NO: 41558 - protein, 9 aa, synthetic construct
GGTGNDGVY

SEQ ID NO: 41559 - protein, 9 aa, synthetic construct
GGTGNDGYR

SEQ ID NO: 41560 - protein, 9 aa, synthetic construct
GGTGNDGYY

SEQ ID NO: 41561 - protein, 9 aa, synthetic construct
GGTGNDHAW

SEQ ID NO: 41562 - protein, 9 aa, synthetic construct
GGTGNDHIY

SEQ ID NO: 41563 - protein, 9 aa, synthetic construct
GGTGNDHLE

SEQ ID NO: 41564 - protein, 9 aa, synthetic construct
GGTGNDHLK

SEQ ID NO: 41565 - protein, 9 aa, synthetic construct
GGTGNDKLV

SEQ ID NO: 41566 - protein, 9 aa, synthetic construct
GGTGNDKMN

SEQ ID NO: 41567 - protein, 9 aa, synthetic construct
GGTGNDKMR

SEQ ID NO: 41568 - protein, 9 aa, synthetic construct
GGTGNDQIK

SEQ ID NO: 41569 - protein, 9 aa, synthetic construct
GGTGNDNLK

SEQ ID NO: 41570 - protein, 9 aa, synthetic construct
GGTGNDNLQ

SEQ ID NO: 41571 - protein, 9 aa, synthetic construct
GGTGNDNLR

SEQ ID NO: 41572 - protein, 9 aa, synthetic construct
GGTGNDNLV

SEQ ID NO: 41573 - protein, 9 aa, synthetic construct
GGTGNDNME

SEQ ID NO: 41574 - protein, 9 aa, synthetic construct
GGTGNDNMQ

SEQ ID NO: 41575 - protein, 9 aa, synthetic construct
GGTGNDNYL

SEQ ID NO: 41576 - protein, 9 aa, synthetic construct
GGTGNDNYV

SEQ ID NO: 41577 - protein, 9 aa, synthetic construct
GGTGNDQAV

SEQ ID NO: 41578 - protein, 9 aa, synthetic construct
GGTGNDQFI

SEQ ID NO: 41579 - protein, 9 aa, synthetic construct
GGTGNDQFV

SEQ ID NO: 41580 - protein, 9 aa, synthetic construct
GGTGNDQIF

SEQ ID NO: 41581 - protein, 9 aa, synthetic construct
GGTGNDQIG

SEQ ID NO: 41582 - protein, 9 aa, synthetic construct
GGTGNDQIL

SEQ ID NO: 41583 - protein, 9 aa, synthetic construct
GGTGNDNLD

SEQ ID NO: 41584 - protein, 9 aa, synthetic construct
GGTGNDQIV

SEQ ID NO: 41585 - protein, 9 aa, synthetic construct
GGTGNDQLL

SEQ ID NO: 41586 - protein, 9 aa, synthetic construct
GGTGNDQLM

SEQ ID NO: 41587 - protein, 9 aa, synthetic construct
GGTGNDQLV

SEQ ID NO: 41588 - protein, 9 aa, synthetic construct
GGTGNDQMF

SEQ ID NO: 41589 - protein, 9 aa, synthetic construct
GGTGNDQMI

SEQ ID NO: 41590 - protein, 9 aa, synthetic construct
GGTGNDQMN

SEQ ID NO: 41591 - protein, 9 aa, synthetic construct
GGTGNDQMW

SEQ ID NO: 41592 - protein, 9 aa, synthetic construct
GGTGNDQVY

SEQ ID NO: 41593 - protein, 9 aa, synthetic construct
GGTGNDQYT

SEQ ID NO: 41594 - protein, 9 aa, synthetic construct
GGTGNDRAS

SEQ ID NO: 41595 - protein, 9 aa, synthetic construct
GGTGNDRAV

SEQ ID NO: 41596 - protein, 9 aa, synthetic construct
GGTGNDRAY

SEQ ID NO: 41597 - protein, 9 aa, synthetic construct
GGTGNDNLH

SEQ ID NO: 41598 - protein, 9 aa, synthetic construct
GGTGNDNIW

SEQ ID NO: 41599 - protein, 9 aa, synthetic construct
GGTGNDKVF

SEQ ID NO: 41600 - protein, 9 aa, synthetic construct
GGTGNDLVT

SEQ ID NO: 41601 - protein, 9 aa, synthetic construct
GGTGNDKYV

SEQ ID NO: 41602 - protein, 9 aa, synthetic construct
GGTGNDLAS

SEQ ID NO: 41603 - protein, 9 aa, synthetic construct
GGTGNDLIF

SEQ ID NO: 41604 - protein, 9 aa, synthetic construct
GGTGNDLIS

SEQ ID NO: 41605 - protein, 9 aa, synthetic construct
GGTGNDLLG

SEQ ID NO: 41606 - protein, 9 aa, synthetic construct
GGTGNDLLM

SEQ ID NO: 41607 - protein, 9 aa, synthetic construct
GGTGNDLMF

SEQ ID NO: 41608 - protein, 9 aa, synthetic construct
GGTGNDLMG

SEQ ID NO: 41609 - protein, 9 aa, synthetic construct
GGTGNDLMK

SEQ ID NO: 41610 - protein, 9 aa, synthetic construct
GGTGNDLMM

SEQ ID NO: 41611 - protein, 9 aa, synthetic construct
GGTGNDLMS

SEQ ID NO: 41612 - protein, 9 aa, synthetic construct
GGTGNDLVF

SEQ ID NO: 41613 - protein, 9 aa, synthetic construct
GGTGNDLVN

SEQ ID NO: 41614 - protein, 9 aa, synthetic construct
GGTGNDMFD

SEQ ID NO: 41615 - protein, 9 aa, synthetic construct
GGTGNDNIS

SEQ ID NO: 41616 - protein, 9 aa, synthetic construct
GGTGNDMIG

SEQ ID NO: 41617 - protein, 9 aa, synthetic construct
GGTGNDMIS

SEQ ID NO: 41618 - protein, 9 aa, synthetic construct
GGTGNDMLG

SEQ ID NO: 41619 - protein, 9 aa, synthetic construct
GGTGNDMLR

SEQ ID NO: 41620 - protein, 9 aa, synthetic construct
GGTGNDMLW

SEQ ID NO: 41621 - protein, 9 aa, synthetic construct
GGTGNDMMS

SEQ ID NO: 41622 - protein, 9 aa, synthetic construct
GGTGNDMMV

SEQ ID NO: 41623 - protein, 9 aa, synthetic construct
GGTGNDMVD

SEQ ID NO: 41624 - protein, 9 aa, synthetic construct
GGTGNDMVI

SEQ ID NO: 41625 - protein, 9 aa, synthetic construct
GGTGNDMYL

SEQ ID NO: 41626 - protein, 9 aa, synthetic construct
GGTGNDNIA

SEQ ID NO: 41627 - protein, 9 aa, synthetic construct
GGTGNDNIH

SEQ ID NO: 41628 - protein, 9 aa, synthetic construct
GGTGNDNII

SEQ ID NO: 41629 - protein, 9 aa, synthetic construct
GGTGQDEIN

SEQ ID NO: 41630 - protein, 9 aa, synthetic construct
GGTGQDFIF

SEQ ID NO: 41631 - protein, 9 aa, synthetic construct
GGTGFDFAS

SEQ ID NO: 41632 - protein, 9 aa, synthetic construct
GGTGRDVLM

SEQ ID NO: 41633 - protein, 9 aa, synthetic construct
GGTGRDSLW

SEQ ID NO: 41634 - protein, 9 aa, synthetic construct
GGTGRDSLY

SEQ ID NO: 41635 - protein, 9 aa, synthetic construct
GGTGRDSVF

SEQ ID NO: 41636 - protein, 9 aa, synthetic construct
GGTGRDSVS

SEQ ID NO: 41637 - protein, 9 aa, synthetic construct
GGTGRDTFA

SEQ ID NO: 41638 - protein, 9 aa, synthetic construct
GGTGRDTFE

SEQ ID NO: 41639 - protein, 9 aa, synthetic construct
GGTGRDTFF

SEQ ID NO: 41640 - protein, 9 aa, synthetic construct
GGTGRDTFI

SEQ ID NO: 41641 - protein, 9 aa, synthetic construct
GGTGRDTFQ

SEQ ID NO: 41642 - protein, 9 aa, synthetic construct
GGTGRDTIA

SEQ ID NO: 41643 - protein, 9 aa, synthetic construct
GGTGRDTIE

SEQ ID NO: 41644 - protein, 9 aa, synthetic construct
GGTGRDTIR

SEQ ID NO: 41645 - protein, 9 aa, synthetic construct
GGTGRDTIT

SEQ ID NO: 41646 - protein, 9 aa, synthetic construct
GGTGRDTLK

SEQ ID NO: 41647 - protein, 9 aa, synthetic construct
GGTGRDTLM

SEQ ID NO: 41648 - protein, 9 aa, synthetic construct
GGTGRDTLW

SEQ ID NO: 41649 - protein, 9 aa, synthetic construct
GGTGRDTMN

SEQ ID NO: 41650 - protein, 9 aa, synthetic construct
GGTGRDTVI

SEQ ID NO: 41651 - protein, 9 aa, synthetic construct
GGTGRDTVK

SEQ ID NO: 41652 - protein, 9 aa, synthetic construct
GGTGRDTVL

SEQ ID NO: 41653 - protein, 9 aa, synthetic construct
GGTGRDTYV

SEQ ID NO: 41654 - protein, 9 aa, synthetic construct
GGTGRDTYY

SEQ ID NO: 41655 - protein, 9 aa, synthetic construct
GGTGRDVAD

SEQ ID NO: 41656 - protein, 9 aa, synthetic construct
GGTGRDVFI

SEQ ID NO: 41657 - protein, 9 aa, synthetic construct
GGTGRDVIG

SEQ ID NO: 41658 - protein, 9 aa, synthetic construct
GGTGRDVII

SEQ ID NO: 41659 - protein, 9 aa, synthetic construct
GGTGRDVIR

SEQ ID NO: 41660 - protein, 9 aa, synthetic construct
GGTGRDVIT

SEQ ID NO: 41661 - protein, 9 aa, synthetic construct
GGTGRDVIY

SEQ ID NO: 41662 - protein, 9 aa, synthetic construct
GGTGRDSLA

SEQ ID NO: 41663 - protein, 9 aa, synthetic construct
GGTGRDSFA

SEQ ID NO: 41664 - protein, 9 aa, synthetic construct
GGTGRDSAH

SEQ ID NO: 41665 - protein, 9 aa, synthetic construct
GGTGRDNLY

SEQ ID NO: 41666 - protein, 9 aa, synthetic construct
GGTGRDLMG

SEQ ID NO: 41667 - protein, 9 aa, synthetic construct
GGTGRDLMQ

SEQ ID NO: 41668 - protein, 9 aa, synthetic construct
GGTGRDLVD

SEQ ID NO: 41669 - protein, 9 aa, synthetic construct
GGTGRDLVN

SEQ ID NO: 41670 - protein, 9 aa, synthetic construct
GGTGRDLVS

SEQ ID NO: 41671 - protein, 9 aa, synthetic construct
GGTGRDLYD

SEQ ID NO: 41672 - protein, 9 aa, synthetic construct
GGTGRDMIF

SEQ ID NO: 41673 - protein, 9 aa, synthetic construct
GGTGRDMLF

SEQ ID NO: 41674 - protein, 9 aa, synthetic construct
GGTGRDMLL

SEQ ID NO: 41675 - protein, 9 aa, synthetic construct
GGTGRDMLR

SEQ ID NO: 41676 - protein, 9 aa, synthetic construct
GGTGRDMVT

SEQ ID NO: 41677 - protein, 9 aa, synthetic construct
GGTGRDNIL

SEQ ID NO: 41678 - protein, 9 aa, synthetic construct
GGTGRDNLQ

SEQ ID NO: 41679 - protein, 9 aa, synthetic construct
GGTGRDQID

SEQ ID NO: 41680 - protein, 9 aa, synthetic construct
GGTGRDRVD

SEQ ID NO: 41681 - protein, 9 aa, synthetic construct
GGTGRDQIF

SEQ ID NO: 41682 - protein, 9 aa, synthetic construct
GGTGRDQLL

SEQ ID NO: 41683 - protein, 9 aa, synthetic construct
GGTGRDQLR

SEQ ID NO: 41684 - protein, 9 aa, synthetic construct
GGTGRDQLS

SEQ ID NO: 41685 - protein, 9 aa, synthetic construct
GGTGRDQLT

SEQ ID NO: 41686 - protein, 9 aa, synthetic construct
GGTGRDRFY

SEQ ID NO: 41687 - protein, 9 aa, synthetic construct
GGTGRDRIM

SEQ ID NO: 41688 - protein, 9 aa, synthetic construct
GGTGRDRLE

SEQ ID NO: 41689 - protein, 9 aa, synthetic construct
GGTGRDRLR

SEQ ID NO: 41690 - protein, 9 aa, synthetic construct
GGTGRDRLS

SEQ ID NO: 41691 - protein, 9 aa, synthetic construct
GGTGRDRME

SEQ ID NO: 41692 - protein, 9 aa, synthetic construct
GGTGRDRMF

SEQ ID NO: 41693 - protein, 9 aa, synthetic construct
GGTGRDRMQ

SEQ ID NO: 41694 - protein, 9 aa, synthetic construct
GGTGRDVLF

SEQ ID NO: 41695 - protein, 9 aa, synthetic construct
GGTGRDVLQ

SEQ ID NO: 41696 - protein, 9 aa, synthetic construct
GGTGQDFIY

SEQ ID NO: 41697 - protein, 9 aa, synthetic construct
GGTGRDVMR

SEQ ID NO: 41698 - protein, 9 aa, synthetic construct
GGTGSDEVS

SEQ ID NO: 41699 - protein, 9 aa, synthetic construct
GGTGSDEVY

SEQ ID NO: 41700 - protein, 9 aa, synthetic construct
GGTGSDFAN

SEQ ID NO: 41701 - protein, 9 aa, synthetic construct
GGTGSDFIV

SEQ ID NO: 41702 - protein, 9 aa, synthetic construct
GGTGSDFLD

SEQ ID NO: 41703 - protein, 9 aa, synthetic construct
GGTGSDFLE

SEQ ID NO: 41704 - protein, 9 aa, synthetic construct
GGTGSDFLS

SEQ ID NO: 41705 - protein, 9 aa, synthetic construct
GGTGSDFLW

SEQ ID NO: 41706 - protein, 9 aa, synthetic construct
GGTGSDFLY

SEQ ID NO: 41707 - protein, 9 aa, synthetic construct
GGTGSDGLR

SEQ ID NO: 41708 - protein, 9 aa, synthetic construct
GGTGSDHFI

SEQ ID NO: 41709 - protein, 9 aa, synthetic construct
GGTGSDHFV

SEQ ID NO: 41710 - protein, 9 aa, synthetic construct
GGTGSDHIN

SEQ ID NO: 41711 - protein, 9 aa, synthetic construct
GGTGSDHLF

SEQ ID NO: 41712 - protein, 9 aa, synthetic construct
GGTGSDHLK

SEQ ID NO: 41713 - protein, 9 aa, synthetic construct
GGTGSDHYH

SEQ ID NO: 41714 - protein, 9 aa, synthetic construct
GGTGSDIFA

SEQ ID NO: 41715 - protein, 9 aa, synthetic construct
GGTGSDIFI

SEQ ID NO: 41716 - protein, 9 aa, synthetic construct
GGTGSDIFQ

SEQ ID NO: 41717 - protein, 9 aa, synthetic construct
GGTGSDIIA

SEQ ID NO: 41718 - protein, 9 aa, synthetic construct
GGTGSDIIY

SEQ ID NO: 41719 - protein, 9 aa, synthetic construct
GGTGSDILD

SEQ ID NO: 41720 - protein, 9 aa, synthetic construct
GGTGSDILL

SEQ ID NO: 41721 - protein, 9 aa, synthetic construct
GGTGSDIMT

SEQ ID NO: 41722 - protein, 9 aa, synthetic construct
GGTGSDIMV

SEQ ID NO: 41723 - protein, 9 aa, synthetic construct
GGTGSDIMY

SEQ ID NO: 41724 - protein, 9 aa, synthetic construct
GGTGSDIVE

SEQ ID NO: 41725 - protein, 9 aa, synthetic construct
GGTGSDIVS

SEQ ID NO: 41726 - protein, 9 aa, synthetic construct
GGTGSDIVT

SEQ ID NO: 41727 - protein, 9 aa, synthetic construct
GGTGSDEMF

SEQ ID NO: 41728 - protein, 9 aa, synthetic construct
GGTGSDELL

SEQ ID NO: 41729 - protein, 9 aa, synthetic construct
GGTGSDEIH

SEQ ID NO: 41730 - protein, 9 aa, synthetic construct
GGTGRDYLW

SEQ ID NO: 41731 - protein, 9 aa, synthetic construct
GGTGRDVMS

SEQ ID NO: 41732 - protein, 9 aa, synthetic construct
GGTGRDVYH

SEQ ID NO: 41733 - protein, 9 aa, synthetic construct
GGTGRDVYV

SEQ ID NO: 41734 - protein, 9 aa, synthetic construct
GGTGRDVYY

SEQ ID NO: 41735 - protein, 9 aa, synthetic construct
GGTGRDWLF

SEQ ID NO: 41736 - protein, 9 aa, synthetic construct
GGTGRDWLL

SEQ ID NO: 41737 - protein, 9 aa, synthetic construct
GGTGRDWLY

SEQ ID NO: 41738 - protein, 9 aa, synthetic construct
GGTGRDWMF

SEQ ID NO: 41739 - protein, 9 aa, synthetic construct
GGTGRDWMV

SEQ ID NO: 41740 - protein, 9 aa, synthetic construct
GGTGRDYLA

SEQ ID NO: 41741 - protein, 9 aa, synthetic construct
GGTGRDYLE

SEQ ID NO: 41742 - protein, 9 aa, synthetic construct
GGTGRDYLF

SEQ ID NO: 41743 - protein, 9 aa, synthetic construct
GGTGRDYLN

SEQ ID NO: 41744 - protein, 9 aa, synthetic construct
GGTGRDYLY

SEQ ID NO: 41745 - protein, 9 aa, synthetic construct
GGTGSDEFV

SEQ ID NO: 41746 - protein, 9 aa, synthetic construct
GGTGSDAIG

SEQ ID NO: 41747 - protein, 9 aa, synthetic construct
GGTGSDALA

SEQ ID NO: 41748 - protein, 9 aa, synthetic construct
GGTGSDALD

SEQ ID NO: 41749 - protein, 9 aa, synthetic construct
GGTGSDALF

SEQ ID NO: 41750 - protein, 9 aa, synthetic construct
GGTGSDAVD

SEQ ID NO: 41751 - protein, 9 aa, synthetic construct
GGTGSDCLF

SEQ ID NO: 41752 - protein, 9 aa, synthetic construct
GGTGSDDID

SEQ ID NO: 41753 - protein, 9 aa, synthetic construct
GGTGSDDLA

SEQ ID NO: 41754 - protein, 9 aa, synthetic construct
GGTGSDDLN

SEQ ID NO: 41755 - protein, 9 aa, synthetic construct
GGTGSDDLS

SEQ ID NO: 41756 - protein, 9 aa, synthetic construct
GGTGSDDLT

SEQ ID NO: 41757 - protein, 9 aa, synthetic construct
GGTGSDDLY

SEQ ID NO: 41758 - protein, 9 aa, synthetic construct
GGTGSDEFH

SEQ ID NO: 41759 - protein, 9 aa, synthetic construct
GGTGRDLLW

SEQ ID NO: 41760 - protein, 9 aa, synthetic construct
GGTGRDLLR

SEQ ID NO: 41761 - protein, 9 aa, synthetic construct
GGTGRDLLK

SEQ ID NO: 41762 - protein, 9 aa, synthetic construct
GGTGRDLLF

SEQ ID NO: 41763 - protein, 9 aa, synthetic construct
GGTGQDRLV

SEQ ID NO: 41764 - protein, 9 aa, synthetic construct
GGTGQDRLY

SEQ ID NO: 41765 - protein, 9 aa, synthetic construct
GGTGQDRMW

SEQ ID NO: 41766 - protein, 9 aa, synthetic construct
GGTGQDRYV

SEQ ID NO: 41767 - protein, 9 aa, synthetic construct
GGTGQDSLW

SEQ ID NO: 41768 - protein, 9 aa, synthetic construct
GGTGQDSMS

SEQ ID NO: 41769 - protein, 9 aa, synthetic construct
GGTGQDTAD

SEQ ID NO: 41770 - protein, 9 aa, synthetic construct
GGTGQDTFL

SEQ ID NO: 41771 - protein, 9 aa, synthetic construct
GGTGQDTFV

SEQ ID NO: 41772 - protein, 9 aa, synthetic construct
GGTGQDTFY

SEQ ID NO: 41773 - protein, 9 aa, synthetic construct
GGTGQDTIE

SEQ ID NO: 41774 - protein, 9 aa, synthetic construct
GGTGQDTLK

SEQ ID NO: 41775 - protein, 9 aa, synthetic construct
GGTGQDTLM

SEQ ID NO: 41776 - protein, 9 aa, synthetic construct
GGTGQDTLP

SEQ ID NO: 41777 - protein, 9 aa, synthetic construct
GGTGQDTLR

SEQ ID NO: 41778 - protein, 9 aa, synthetic construct
GGTGQDTLW

SEQ ID NO: 41779 - protein, 9 aa, synthetic construct
GGTGQDTMI

SEQ ID NO: 41780 - protein, 9 aa, synthetic construct
GGTGQDTML

SEQ ID NO: 41781 - protein, 9 aa, synthetic construct
GGTGQDTVH

SEQ ID NO: 41782 - protein, 9 aa, synthetic construct
GGTGQDTVY

SEQ ID NO: 41783 - protein, 9 aa, synthetic construct
GGTGQDTYI

SEQ ID NO: 41784 - protein, 9 aa, synthetic construct
GGTGQDVFR

SEQ ID NO: 41785 - protein, 9 aa, synthetic construct
GGTGQDVIA

SEQ ID NO: 41786 - protein, 9 aa, synthetic construct
GGTGQDVIE

SEQ ID NO: 41787 - protein, 9 aa, synthetic construct
GGTGQDVIR

SEQ ID NO: 41788 - protein, 9 aa, synthetic construct
GGTGQDVLI

SEQ ID NO: 41789 - protein, 9 aa, synthetic construct
GGTGQDVLN

SEQ ID NO: 41790 - protein, 9 aa, synthetic construct
GGTGQDVLQ

SEQ ID NO: 41791 - protein, 9 aa, synthetic construct
GGTGQDVLR

SEQ ID NO: 41792 - protein, 9 aa, synthetic construct
GGTGQDRLI

SEQ ID NO: 41793 - protein, 9 aa, synthetic construct
GGTGQDRIY

SEQ ID NO: 41794 - protein, 9 aa, synthetic construct
GGTGQDRIN

SEQ ID NO: 41795 - protein, 9 aa, synthetic construct
GGTGQDLLF

SEQ ID NO: 41796 - protein, 9 aa, synthetic construct
GGTGQDFLS

SEQ ID NO: 41797 - protein, 9 aa, synthetic construct
GGTGQDFLY

SEQ ID NO: 41798 - protein, 9 aa, synthetic construct
GGTGQDFVH

SEQ ID NO: 41799 - protein, 9 aa, synthetic construct
GGTGQDGLW

SEQ ID NO: 41800 - protein, 9 aa, synthetic construct
GGTGQDGVL

SEQ ID NO: 41801 - protein, 9 aa, synthetic construct
GGTGQDHLF

SEQ ID NO: 41802 - protein, 9 aa, synthetic construct
GGTGQDHLV

SEQ ID NO: 41803 - protein, 9 aa, synthetic construct
GGTGQDIID

SEQ ID NO: 41804 - protein, 9 aa, synthetic construct
GGTGQDILL

SEQ ID NO: 41805 - protein, 9 aa, synthetic construct
GGTGQDILS

SEQ ID NO: 41806 - protein, 9 aa, synthetic construct
GGTGQDLID

SEQ ID NO: 41807 - protein, 9 aa, synthetic construct
GGTGQDLIY

SEQ ID NO: 41808 - protein, 9 aa, synthetic construct
GGTGQDLLD

SEQ ID NO: 41809 - protein, 9 aa, synthetic construct
GGTGQDLLN

SEQ ID NO: 41810 - protein, 9 aa, synthetic construct
GGTGQDRIL

SEQ ID NO: 41811 - protein, 9 aa, synthetic construct
GGTGQDLLV

SEQ ID NO: 41812 - protein, 9 aa, synthetic construct
GGTGQDLLY

SEQ ID NO: 41813 - protein, 9 aa, synthetic construct
GGTGQDMAV

SEQ ID NO: 41814 - protein, 9 aa, synthetic construct
GGTGQDMLR

SEQ ID NO: 41815 - protein, 9 aa, synthetic construct
GGTGQDMLS

SEQ ID NO: 41816 - protein, 9 aa, synthetic construct
GGTGQDNLF

SEQ ID NO: 41817 - protein, 9 aa, synthetic construct
GGTGQDNLL

SEQ ID NO: 41818 - protein, 9 aa, synthetic construct
GGTGQDNVD

SEQ ID NO: 41819 - protein, 9 aa, synthetic construct
GGTGQDQIN

SEQ ID NO: 41820 - protein, 9 aa, synthetic construct
GGTGQDQIY

SEQ ID NO: 41821 - protein, 9 aa, synthetic construct
GGTGQDQLY

SEQ ID NO: 41822 - protein, 9 aa, synthetic construct
GGTGQDQMI

SEQ ID NO: 41823 - protein, 9 aa, synthetic construct
GGTGQDRIE

SEQ ID NO: 41824 - protein, 9 aa, synthetic construct
GGTGQDVLS

SEQ ID NO: 41825 - protein, 9 aa, synthetic construct
GGTGQDWID

SEQ ID NO: 41826 - protein, 9 aa, synthetic construct
GGTGQDWIS

SEQ ID NO: 41827 - protein, 9 aa, synthetic construct
GGTGRDIVD

SEQ ID NO: 41828 - protein, 9 aa, synthetic construct
GGTGRDHLN

SEQ ID NO: 41829 - protein, 9 aa, synthetic construct
GGTGRDHLW

SEQ ID NO: 41830 - protein, 9 aa, synthetic construct
GGTGRDHLY

SEQ ID NO: 41831 - protein, 9 aa, synthetic construct
GGTGRDIFA

SEQ ID NO: 41832 - protein, 9 aa, synthetic construct
GGTGRDIFL

SEQ ID NO: 41833 - protein, 9 aa, synthetic construct
GGTGRDIFR

SEQ ID NO: 41834 - protein, 9 aa, synthetic construct
GGTGRDILD

SEQ ID NO: 41835 - protein, 9 aa, synthetic construct
GGTGRDILG

SEQ ID NO: 41836 - protein, 9 aa, synthetic construct
GGTGRDILI

SEQ ID NO: 41837 - protein, 9 aa, synthetic construct
GGTGRDILK

SEQ ID NO: 41838 - protein, 9 aa, synthetic construct
GGTGRDILR

SEQ ID NO: 41839 - protein, 9 aa, synthetic construct
GGTGRDIMT

SEQ ID NO: 41840 - protein, 9 aa, synthetic construct
GGTGRDIMV

SEQ ID NO: 41841 - protein, 9 aa, synthetic construct
GGTGRDIVN

SEQ ID NO: 41842 - protein, 9 aa, synthetic construct
GGTGRDHLE

SEQ ID NO: 41843 - protein, 9 aa, synthetic construct
GGTGRDIYV

SEQ ID NO: 41844 - protein, 9 aa, synthetic construct
GGTGRDKLA

SEQ ID NO: 41845 - protein, 9 aa, synthetic construct
GGTGRDKLD

SEQ ID NO: 41846 - protein, 9 aa, synthetic construct
GGTGRDKLK

SEQ ID NO: 41847 - protein, 9 aa, synthetic construct
GGTGRDKLY

SEQ ID NO: 41848 - protein, 9 aa, synthetic construct
GGTGRDKMF

SEQ ID NO: 41849 - protein, 9 aa, synthetic construct
GGTGRDKMI

SEQ ID NO: 41850 - protein, 9 aa, synthetic construct
GGTGRDKMY

SEQ ID NO: 41851 - protein, 9 aa, synthetic construct
GGTGRDLAY

SEQ ID NO: 41852 - protein, 9 aa, synthetic construct
GGTGRDLFV

SEQ ID NO: 41853 - protein, 9 aa, synthetic construct
GGTGRDLIG

SEQ ID NO: 41854 - protein, 9 aa, synthetic construct
GGTGRDLIH

SEQ ID NO: 41855 - protein, 9 aa, synthetic construct
GGTGRDLIY

SEQ ID NO: 41856 - protein, 9 aa, synthetic construct
GGTGRDHLK

SEQ ID NO: 41857 - protein, 9 aa, synthetic construct
GGTGRDHLD

SEQ ID NO: 41858 - protein, 9 aa, synthetic construct
GGTGQDWLR

SEQ ID NO: 41859 - protein, 9 aa, synthetic construct
GGTGRDDLY

SEQ ID NO: 41860 - protein, 9 aa, synthetic construct
GGTGQDYFY

SEQ ID NO: 41861 - protein, 9 aa, synthetic construct
GGTGQDYLA

SEQ ID NO: 41862 - protein, 9 aa, synthetic construct
GGTGQDYLN

SEQ ID NO: 41863 - protein, 9 aa, synthetic construct
GGTGQDYLS

SEQ ID NO: 41864 - protein, 9 aa, synthetic construct
GGTGQDYMN

SEQ ID NO: 41865 - protein, 9 aa, synthetic construct
GGTGRDALF

SEQ ID NO: 41866 - protein, 9 aa, synthetic construct
GGTGRDALH

SEQ ID NO: 41867 - protein, 9 aa, synthetic construct
GGTGRDALI

SEQ ID NO: 41868 - protein, 9 aa, synthetic construct
GGTGRDALR

SEQ ID NO: 41869 - protein, 9 aa, synthetic construct
GGTGRDALY

SEQ ID NO: 41870 - protein, 9 aa, synthetic construct
GGTGRDAMT

SEQ ID NO: 41871 - protein, 9 aa, synthetic construct
GGTGRDDIE

SEQ ID NO: 41872 - protein, 9 aa, synthetic construct
GGTGRDDLG

SEQ ID NO: 41873 - protein, 9 aa, synthetic construct
GGTGRDDMQ

SEQ ID NO: 41874 - protein, 9 aa, synthetic construct
GGTGRDHFV

SEQ ID NO: 41875 - protein, 9 aa, synthetic construct
GGTGRDDVA

SEQ ID NO: 41876 - protein, 9 aa, synthetic construct
GGTGRDEFV

SEQ ID NO: 41877 - protein, 9 aa, synthetic construct
GGTGRDELF

SEQ ID NO: 41878 - protein, 9 aa, synthetic construct
GGTGRDELH

SEQ ID NO: 41879 - protein, 9 aa, synthetic construct
GGTGRDELR

SEQ ID NO: 41880 - protein, 9 aa, synthetic construct
GGTGRDELV

SEQ ID NO: 41881 - protein, 9 aa, synthetic construct
GGTGRDELW

SEQ ID NO: 41882 - protein, 9 aa, synthetic construct
GGTGRDFIF

SEQ ID NO: 41883 - protein, 9 aa, synthetic construct
GGTGRDFLF

SEQ ID NO: 41884 - protein, 9 aa, synthetic construct
GGTGRDFLR

SEQ ID NO: 41885 - protein, 9 aa, synthetic construct
GGTGRDFLV

SEQ ID NO: 41886 - protein, 9 aa, synthetic construct
GGTGRDFMT

SEQ ID NO: 41887 - protein, 9 aa, synthetic construct
GGTGRDHAY

SEQ ID NO: 41888 - protein, 9 aa, synthetic construct
GGTGNDEVY

SEQ ID NO: 41889 - protein, 9 aa, synthetic construct
GGTGNDEVS

SEQ ID NO: 41890 - protein, 9 aa, synthetic construct
GGTGNDEVL

SEQ ID NO: 41891 - protein, 9 aa, synthetic construct
GGTGHDSLT

SEQ ID NO: 41892 - protein, 9 aa, synthetic construct
GGTGHDKLY

SEQ ID NO: 41893 - protein, 9 aa, synthetic construct
GGTGHDLAF

SEQ ID NO: 41894 - protein, 9 aa, synthetic construct
GGTGHDLIE

SEQ ID NO: 41895 - protein, 9 aa, synthetic construct
GGTGHDLIH

SEQ ID NO: 41896 - protein, 9 aa, synthetic construct
GGTGHDLLE

SEQ ID NO: 41897 - protein, 9 aa, synthetic construct
GGTGHDLLN

SEQ ID NO: 41898 - protein, 9 aa, synthetic construct
GGTGHDLMD

SEQ ID NO: 41899 - protein, 9 aa, synthetic construct
GGTGHDMLN

SEQ ID NO: 41900 - protein, 9 aa, synthetic construct
GGTGHDNLE

SEQ ID NO: 41901 - protein, 9 aa, synthetic construct
GGTGHDNLL

SEQ ID NO: 41902 - protein, 9 aa, synthetic construct
GGTGHDQFV

SEQ ID NO: 41903 - protein, 9 aa, synthetic construct
GGTGHDQIF

SEQ ID NO: 41904 - protein, 9 aa, synthetic construct
GGTGHDRAA

SEQ ID NO: 41905 - protein, 9 aa, synthetic construct
GGTGHDRFY

SEQ ID NO: 41906 - protein, 9 aa, synthetic construct
GGTGHDRIF

SEQ ID NO: 41907 - protein, 9 aa, synthetic construct
GGTGHDRIL

SEQ ID NO: 41908 - protein, 9 aa, synthetic construct
GGTGHDRIV

SEQ ID NO: 41909 - protein, 9 aa, synthetic construct
GGTGHDRLA

SEQ ID NO: 41910 - protein, 9 aa, synthetic construct
GGTGHDRLR

SEQ ID NO: 41911 - protein, 9 aa, synthetic construct
GGTGHDRLS

SEQ ID NO: 41912 - protein, 9 aa, synthetic construct
GGTGHDRLV

SEQ ID NO: 41913 - protein, 9 aa, synthetic construct
GGTGHDRLW

SEQ ID NO: 41914 - protein, 9 aa, synthetic construct
GGTGHDRMF

SEQ ID NO: 41915 - protein, 9 aa, synthetic construct
GGTGHDRMH

SEQ ID NO: 41916 - protein, 9 aa, synthetic construct
GGTGHDRYQ

SEQ ID NO: 41917 - protein, 9 aa, synthetic construct
GGTGHDSFV

SEQ ID NO: 41918 - protein, 9 aa, synthetic construct
GGTGHDSIL

SEQ ID NO: 41919 - protein, 9 aa, synthetic construct
GGTGHDSLA

SEQ ID NO: 41920 - protein, 9 aa, synthetic construct
GGTGHDSLD

SEQ ID NO: 41921 - protein, 9 aa, synthetic construct
GGTGHDIMY

SEQ ID NO: 41922 - protein, 9 aa, synthetic construct
GGTGHDIMM

SEQ ID NO: 41923 - protein, 9 aa, synthetic construct
GGTGHDIMF

SEQ ID NO: 41924 - protein, 9 aa, synthetic construct
GGTGHDALN

SEQ ID NO: 41925 - protein, 9 aa, synthetic construct
GGTGGDWLF

SEQ ID NO: 41926 - protein, 9 aa, synthetic construct
GGTGGDWLS

SEQ ID NO: 41927 - protein, 9 aa, synthetic construct
GGTGGDYIE

SEQ ID NO: 41928 - protein, 9 aa, synthetic construct
GGTGGDYLN

SEQ ID NO: 41929 - protein, 9 aa, synthetic construct
GGTGGDYLS

SEQ ID NO: 41930 - protein, 9 aa, synthetic construct
GGTGGDYLW

SEQ ID NO: 41931 - protein, 9 aa, synthetic construct
GGTGHDAAM

SEQ ID NO: 41932 - protein, 9 aa, synthetic construct
GGTGHDAIT

SEQ ID NO: 41933 - protein, 9 aa, synthetic construct
GGTGHDALA

SEQ ID NO: 41934 - protein, 9 aa, synthetic construct
GGTGHDALF

SEQ ID NO: 41935 - protein, 9 aa, synthetic construct
GGTGHDALH

SEQ ID NO: 41936 - protein, 9 aa, synthetic construct
GGTGHDALK

SEQ ID NO: 41937 - protein, 9 aa, synthetic construct
GGTGHDALL

SEQ ID NO: 41938 - protein, 9 aa, synthetic construct
GGTGHDAMN

SEQ ID NO: 41939 - protein, 9 aa, synthetic construct
GGTGHDILV

SEQ ID NO: 41940 - protein, 9 aa, synthetic construct
GGTGHDAMR

SEQ ID NO: 41941 - protein, 9 aa, synthetic construct
GGTGHDDIS

SEQ ID NO: 41942 - protein, 9 aa, synthetic construct
GGTGHDDLF

SEQ ID NO: 41943 - protein, 9 aa, synthetic construct
GGTGHDEAY

SEQ ID NO: 41944 - protein, 9 aa, synthetic construct
GGTGHDELL

SEQ ID NO: 41945 - protein, 9 aa, synthetic construct
GGTGHDELR

SEQ ID NO: 41946 - protein, 9 aa, synthetic construct
GGTGHDFLM

SEQ ID NO: 41947 - protein, 9 aa, synthetic construct
GGTGHDFLR

SEQ ID NO: 41948 - protein, 9 aa, synthetic construct
GGTGHDGMR

SEQ ID NO: 41949 - protein, 9 aa, synthetic construct
GGTGHDHVM

SEQ ID NO: 41950 - protein, 9 aa, synthetic construct
GGTGHDIIH

SEQ ID NO: 41951 - protein, 9 aa, synthetic construct
GGTGHDILF

SEQ ID NO: 41952 - protein, 9 aa, synthetic construct
GGTGHDILI

SEQ ID NO: 41953 - protein, 9 aa, synthetic construct
GGTGHDSLS

SEQ ID NO: 41954 - protein, 9 aa, synthetic construct
GGTGHDSLY

SEQ ID NO: 41955 - protein, 9 aa, synthetic construct
GGTGNDEVI

SEQ ID NO: 41956 - protein, 9 aa, synthetic construct
GGTGHDSMG

SEQ ID NO: 41957 - protein, 9 aa, synthetic construct
GGTGIDDLR

SEQ ID NO: 41958 - protein, 9 aa, synthetic construct
GGTGIDDVH

SEQ ID NO: 41959 - protein, 9 aa, synthetic construct
GGTGIDELI

SEQ ID NO: 41960 - protein, 9 aa, synthetic construct
GGTGIDFFN

SEQ ID NO: 41961 - protein, 9 aa, synthetic construct
GGTGIDGIL

SEQ ID NO: 41962 - protein, 9 aa, synthetic construct
GGTGIDIAD

SEQ ID NO: 41963 - protein, 9 aa, synthetic construct
GGTGIDILN

SEQ ID NO: 41964 - protein, 9 aa, synthetic construct
GGTGIDIMD

SEQ ID NO: 41965 - protein, 9 aa, synthetic construct
GGTGIDIMT

SEQ ID NO: 41966 - protein, 9 aa, synthetic construct
GGTGIDIVL

SEQ ID NO: 41967 - protein, 9 aa, synthetic construct
GGTGIDIVN

SEQ ID NO: 41968 - protein, 9 aa, synthetic construct
GGTGIDIVV

SEQ ID NO: 41969 - protein, 9 aa, synthetic construct
GGTGIDKAI

SEQ ID NO: 41970 - protein, 9 aa, synthetic construct
GGTGIDKLV

SEQ ID NO: 41971 - protein, 9 aa, synthetic construct
GGTGIDLFL

SEQ ID NO: 41972 - protein, 9 aa, synthetic construct
GGTGIDLLE

SEQ ID NO: 41973 - protein, 9 aa, synthetic construct
GGTGIDLLT

SEQ ID NO: 41974 - protein, 9 aa, synthetic construct
GGTGIDLVQ

SEQ ID NO: 41975 - protein, 9 aa, synthetic construct
GGTGIDNLT

SEQ ID NO: 41976 - protein, 9 aa, synthetic construct
GGTGIDQLF

SEQ ID NO: 41977 - protein, 9 aa, synthetic construct
GGTGIDQLI

SEQ ID NO: 41978 - protein, 9 aa, synthetic construct
GGTGIDQLL

SEQ ID NO: 41979 - protein, 9 aa, synthetic construct
GGTGIDRAI

SEQ ID NO: 41980 - protein, 9 aa, synthetic construct
GGTGIDRAN

SEQ ID NO: 41981 - protein, 9 aa, synthetic construct
GGTGIDRAQ

SEQ ID NO: 41982 - protein, 9 aa, synthetic construct
GGTGIDRAV

SEQ ID NO: 41983 - protein, 9 aa, synthetic construct
GGTGIDRIL

SEQ ID NO: 41984 - protein, 9 aa, synthetic construct
GGTGIDRLE

SEQ ID NO: 41985 - protein, 9 aa, synthetic construct
GGTGIDRLF

SEQ ID NO: 41986 - protein, 9 aa, synthetic construct
GGTGIDDFV

SEQ ID NO: 41987 - protein, 9 aa, synthetic construct
GGTGIDAMN

SEQ ID NO: 41988 - protein, 9 aa, synthetic construct
GGTGIDAME

SEQ ID NO: 41989 - protein, 9 aa, synthetic construct
GGTGHDVID

SEQ ID NO: 41990 - protein, 9 aa, synthetic construct
GGTGHDSVD

SEQ ID NO: 41991 - protein, 9 aa, synthetic construct
GGTGHDSVR

SEQ ID NO: 41992 - protein, 9 aa, synthetic construct
GGTGHDSVS

SEQ ID NO: 41993 - protein, 9 aa, synthetic construct
GGTGHDTAL

SEQ ID NO: 41994 - protein, 9 aa, synthetic construct
GGTGHDTFV

SEQ ID NO: 41995 - protein, 9 aa, synthetic construct
GGTGHDTIH

SEQ ID NO: 41996 - protein, 9 aa, synthetic construct
GGTGHDTIN

SEQ ID NO: 41997 - protein, 9 aa, synthetic construct
GGTGHDTMD

SEQ ID NO: 41998 - protein, 9 aa, synthetic construct
GGTGHDTMR

SEQ ID NO: 41999 - protein, 9 aa, synthetic construct
GGTGHDTMS

SEQ ID NO: 42000 - protein, 9 aa, synthetic construct
GGTGHDTMY

SEQ ID NO: 42001 - protein, 9 aa, synthetic construct
GGTGHDTVV

SEQ ID NO: 42002 - protein, 9 aa, synthetic construct
GGTGHDVFR

SEQ ID NO: 42003 - protein, 9 aa, synthetic construct
GGTGHDVIS

SEQ ID NO: 42004 - protein, 9 aa, synthetic construct
GGTGIDAMD

SEQ ID NO: 42005 - protein, 9 aa, synthetic construct
GGTGHDVLA

SEQ ID NO: 42006 - protein, 9 aa, synthetic construct
GGTGHDVLC

SEQ ID NO: 42007 - protein, 9 aa, synthetic construct
GGTGHDVLF

SEQ ID NO: 42008 - protein, 9 aa, synthetic construct
GGTGHDWIE

SEQ ID NO: 42009 - protein, 9 aa, synthetic construct
GGTGHDYLI

SEQ ID NO: 42010 - protein, 9 aa, synthetic construct
GGTGHDYLY

SEQ ID NO: 42011 - protein, 9 aa, synthetic construct
GGTGHDYMA

SEQ ID NO: 42012 - protein, 9 aa, synthetic construct
GGTGHDYMR

SEQ ID NO: 42013 - protein, 9 aa, synthetic construct
GGTGHDYYY

SEQ ID NO: 42014 - protein, 9 aa, synthetic construct
GGTGIDALE

SEQ ID NO: 42015 - protein, 9 aa, synthetic construct
GGTGIDALI

SEQ ID NO: 42016 - protein, 9 aa, synthetic construct
GGTGIDALL

SEQ ID NO: 42017 - protein, 9 aa, synthetic construct
GGTGIDALN

SEQ ID NO: 42018 - protein, 9 aa, synthetic construct
GGTGGDWLE

SEQ ID NO: 42019 - protein, 9 aa, synthetic construct
GGTGGDWAS

SEQ ID NO: 42020 - protein, 9 aa, synthetic construct
GGTGGDVYV

SEQ ID NO: 42021 - protein, 9 aa, synthetic construct
GGTGGDVYR

SEQ ID NO: 42022 - protein, 9 aa, synthetic construct
GGTGFDVAS

SEQ ID NO: 42023 - protein, 9 aa, synthetic construct
GGTGFDVAV

SEQ ID NO: 42024 - protein, 9 aa, synthetic construct
GGTGFDVIE

SEQ ID NO: 42025 - protein, 9 aa, synthetic construct
GGTGFDVLD

SEQ ID NO: 42026 - protein, 9 aa, synthetic construct
GGTGFDVLT

SEQ ID NO: 42027 - protein, 9 aa, synthetic construct
GGTGFDYIE

SEQ ID NO: 42028 - protein, 9 aa, synthetic construct
GGTGFDYLS

SEQ ID NO: 42029 - protein, 9 aa, synthetic construct
GGTGGDALE

SEQ ID NO: 42030 - protein, 9 aa, synthetic construct
GGTGGDALI

SEQ ID NO: 42031 - protein, 9 aa, synthetic construct
GGTGGDALT

SEQ ID NO: 42032 - protein, 9 aa, synthetic construct
GGTGGDAMA

SEQ ID NO: 42033 - protein, 9 aa, synthetic construct
GGTGGDDLS

SEQ ID NO: 42034 - protein, 9 aa, synthetic construct
GGTGGDDLW

SEQ ID NO: 42035 - protein, 9 aa, synthetic construct
GGTGGDDLY

SEQ ID NO: 42036 - protein, 9 aa, synthetic construct
GGTGGDEFI

SEQ ID NO: 42037 - protein, 9 aa, synthetic construct
GGTGGDEIW

SEQ ID NO: 42038 - protein, 9 aa, synthetic construct
GGTGGDELF

SEQ ID NO: 42039 - protein, 9 aa, synthetic construct
GGTGGDELL

SEQ ID NO: 42040 - protein, 9 aa, synthetic construct
GGTGGDELS

SEQ ID NO: 42041 - protein, 9 aa, synthetic construct
GGTGGDEVN

SEQ ID NO: 42042 - protein, 9 aa, synthetic construct
GGTGGDFFR

SEQ ID NO: 42043 - protein, 9 aa, synthetic construct
GGTGGDFIE

SEQ ID NO: 42044 - protein, 9 aa, synthetic construct
GGTGGDFIV

SEQ ID NO: 42045 - protein, 9 aa, synthetic construct
GGTGGDFMA

SEQ ID NO: 42046 - protein, 9 aa, synthetic construct
GGTGGDGLE

SEQ ID NO: 42047 - protein, 9 aa, synthetic construct
GGTGGDGLS

SEQ ID NO: 42048 - protein, 9 aa, synthetic construct
GGTGGDILI

SEQ ID NO: 42049 - protein, 9 aa, synthetic construct
GGTGGDILL

SEQ ID NO: 42050 - protein, 9 aa, synthetic construct
GGTGGDILS

SEQ ID NO: 42051 - protein, 9 aa, synthetic construct
GGTGFDTYY

SEQ ID NO: 42052 - protein, 9 aa, synthetic construct
GGTGFDTYI

SEQ ID NO: 42053 - protein, 9 aa, synthetic construct
GGTGFDTVS

SEQ ID NO: 42054 - protein, 9 aa, synthetic construct
GGTGFDQVD

SEQ ID NO: 42055 - protein, 9 aa, synthetic construct
GGTGFDFAV

SEQ ID NO: 42056 - protein, 9 aa, synthetic construct
GGTGFDHLE

SEQ ID NO: 42057 - protein, 9 aa, synthetic construct
GGTGFDIAS

SEQ ID NO: 42058 - protein, 9 aa, synthetic construct
GGTGFDKAV

SEQ ID NO: 42059 - protein, 9 aa, synthetic construct
GGTGFDKLF

SEQ ID NO: 42060 - protein, 9 aa, synthetic construct
GGTGFDKLL

SEQ ID NO: 42061 - protein, 9 aa, synthetic construct
GGTGFDLIF

SEQ ID NO: 42062 - protein, 9 aa, synthetic construct
GGTGFDLLE

SEQ ID NO: 42063 - protein, 9 aa, synthetic construct
GGTGFDLMF

SEQ ID NO: 42064 - protein, 9 aa, synthetic construct
GGTGFDLVS

SEQ ID NO: 42065 - protein, 9 aa, synthetic construct
GGTGFDQLA

SEQ ID NO: 42066 - protein, 9 aa, synthetic construct
GGTGFDQLV

SEQ ID NO: 42067 - protein, 9 aa, synthetic construct
GGTGFDQMS

SEQ ID NO: 42068 - protein, 9 aa, synthetic construct
GGTGFDRIL

SEQ ID NO: 42069 - protein, 9 aa, synthetic construct
GGTGFDTVD

SEQ ID NO: 42070 - protein, 9 aa, synthetic construct
GGTGFDRLV

SEQ ID NO: 42071 - protein, 9 aa, synthetic construct
GGTGFDSIF

SEQ ID NO: 42072 - protein, 9 aa, synthetic construct
GGTGFDSIY

SEQ ID NO: 42073 - protein, 9 aa, synthetic construct
GGTGFDSLS

SEQ ID NO: 42074 - protein, 9 aa, synthetic construct
GGTGFDSLV

SEQ ID NO: 42075 - protein, 9 aa, synthetic construct
GGTGFDSLY

SEQ ID NO: 42076 - protein, 9 aa, synthetic construct
GGTGFDTAD

SEQ ID NO: 42077 - protein, 9 aa, synthetic construct
GGTGFDTAS

SEQ ID NO: 42078 - protein, 9 aa, synthetic construct
GGTGFDTFD

SEQ ID NO: 42079 - protein, 9 aa, synthetic construct
GGTGFDTLF

SEQ ID NO: 42080 - protein, 9 aa, synthetic construct
GGTGFDTLL

SEQ ID NO: 42081 - protein, 9 aa, synthetic construct
GGTGFDTLV

SEQ ID NO: 42082 - protein, 9 aa, synthetic construct
GGTGFDTLY

SEQ ID NO: 42083 - protein, 9 aa, synthetic construct
GGTGGDILV

SEQ ID NO: 42084 - protein, 9 aa, synthetic construct
GGTGGDIVI

SEQ ID NO: 42085 - protein, 9 aa, synthetic construct
GGTGGDKIY

SEQ ID NO: 42086 - protein, 9 aa, synthetic construct
GGTGGDTMT

SEQ ID NO: 42087 - protein, 9 aa, synthetic construct
GGTGGDSIT

SEQ ID NO: 42088 - protein, 9 aa, synthetic construct
GGTGGDSLT

SEQ ID NO: 42089 - protein, 9 aa, synthetic construct
GGTGGDSMG

SEQ ID NO: 42090 - protein, 9 aa, synthetic construct
GGTGGDTAL

SEQ ID NO: 42091 - protein, 9 aa, synthetic construct
GGTGGDTFY

SEQ ID NO: 42092 - protein, 9 aa, synthetic construct
GGTGGDTIA

SEQ ID NO: 42093 - protein, 9 aa, synthetic construct
GGTGGDTID

SEQ ID NO: 42094 - protein, 9 aa, synthetic construct
GGTGGDTIN

SEQ ID NO: 42095 - protein, 9 aa, synthetic construct
GGTGGDTIS

SEQ ID NO: 42096 - protein, 9 aa, synthetic construct
GGTGGDTLG

SEQ ID NO: 42097 - protein, 9 aa, synthetic construct
GGTGGDTLK

SEQ ID NO: 42098 - protein, 9 aa, synthetic construct
GGTGGDTMD

SEQ ID NO: 42099 - protein, 9 aa, synthetic construct
GGTGGDTMS

SEQ ID NO: 42100 - protein, 9 aa, synthetic construct
GGTGGDTMV

SEQ ID NO: 42101 - protein, 9 aa, synthetic construct
GGTGGDRME

SEQ ID NO: 42102 - protein, 9 aa, synthetic construct
GGTGGDTVI

SEQ ID NO: 42103 - protein, 9 aa, synthetic construct
GGTGGDVAV

SEQ ID NO: 42104 - protein, 9 aa, synthetic construct
GGTGGDVFY

SEQ ID NO: 42105 - protein, 9 aa, synthetic construct
GGTGGDVIG

SEQ ID NO: 42106 - protein, 9 aa, synthetic construct
GGTGGDVIY

SEQ ID NO: 42107 - protein, 9 aa, synthetic construct
GGTGGDVLD

SEQ ID NO: 42108 - protein, 9 aa, synthetic construct
GGTGGDVLS

SEQ ID NO: 42109 - protein, 9 aa, synthetic construct
GGTGGDVLV

SEQ ID NO: 42110 - protein, 9 aa, synthetic construct
GGTGGDVLY

SEQ ID NO: 42111 - protein, 9 aa, synthetic construct
GGTGGDVMA

SEQ ID NO: 42112 - protein, 9 aa, synthetic construct
GGTGGDVMD

SEQ ID NO: 42113 - protein, 9 aa, synthetic construct
GGTGGDVMN

SEQ ID NO: 42114 - protein, 9 aa, synthetic construct
GGTGGDVMR

SEQ ID NO: 42115 - protein, 9 aa, synthetic construct
GGTGGDSIH

SEQ ID NO: 42116 - protein, 9 aa, synthetic construct
GGTGGDRLY

SEQ ID NO: 42117 - protein, 9 aa, synthetic construct
GGTGGDKLD

SEQ ID NO: 42118 - protein, 9 aa, synthetic construct
GGTGGDMIT

SEQ ID NO: 42119 - protein, 9 aa, synthetic construct
GGTGGDKLF

SEQ ID NO: 42120 - protein, 9 aa, synthetic construct
GGTGGDKLI

SEQ ID NO: 42121 - protein, 9 aa, synthetic construct
GGTGGDKLQ

SEQ ID NO: 42122 - protein, 9 aa, synthetic construct
GGTGGDKLS

SEQ ID NO: 42123 - protein, 9 aa, synthetic construct
GGTGGDLFR

SEQ ID NO: 42124 - protein, 9 aa, synthetic construct
GGTGGDLLQ

SEQ ID NO: 42125 - protein, 9 aa, synthetic construct
GGTGGDLLR

SEQ ID NO: 42126 - protein, 9 aa, synthetic construct
GGTGGDLLT

SEQ ID NO: 42127 - protein, 9 aa, synthetic construct
GGTGGDLMY

SEQ ID NO: 42128 - protein, 9 aa, synthetic construct
GGTGGDLVI

SEQ ID NO: 42129 - protein, 9 aa, synthetic construct
GGTGGDLVR

SEQ ID NO: 42130 - protein, 9 aa, synthetic construct
GGTGGDLYK

SEQ ID NO: 42131 - protein, 9 aa, synthetic construct
GGTGGDLYL

SEQ ID NO: 42132 - protein, 9 aa, synthetic construct
GGTGGDMLD

SEQ ID NO: 42133 - protein, 9 aa, synthetic construct
GGTGGDRLR

SEQ ID NO: 42134 - protein, 9 aa, synthetic construct
GGTGGDMLE

SEQ ID NO: 42135 - protein, 9 aa, synthetic construct
GGTGGDMLN

SEQ ID NO: 42136 - protein, 9 aa, synthetic construct
GGTGGDMMY

SEQ ID NO: 42137 - protein, 9 aa, synthetic construct
GGTGGDNIL

SEQ ID NO: 42138 - protein, 9 aa, synthetic construct
GGTGGDNIS

SEQ ID NO: 42139 - protein, 9 aa, synthetic construct
GGTGGDNLD

SEQ ID NO: 42140 - protein, 9 aa, synthetic construct
GGTGGDQIW

SEQ ID NO: 42141 - protein, 9 aa, synthetic construct
GGTGGDQMY

SEQ ID NO: 42142 - protein, 9 aa, synthetic construct
GGTGGDRFL

SEQ ID NO: 42143 - protein, 9 aa, synthetic construct
GGTGGDRIF

SEQ ID NO: 42144 - protein, 9 aa, synthetic construct
GGTGGDRIL

SEQ ID NO: 42145 - protein, 9 aa, synthetic construct
GGTGGDRLD

SEQ ID NO: 42146 - protein, 9 aa, synthetic construct
GGTGGDRLI

SEQ ID NO: 42147 - protein, 9 aa, synthetic construct
GGTGIDRLT

SEQ ID NO: 42148 - protein, 9 aa, synthetic construct
GGTGIDRLY

SEQ ID NO: 42149 - protein, 9 aa, synthetic construct
GGTGIDRME

SEQ ID NO: 42150 - protein, 9 aa, synthetic construct
GGTGLDEAY

SEQ ID NO: 42151 - protein, 9 aa, synthetic construct
GGTGLDTAF

SEQ ID NO: 42152 - protein, 9 aa, synthetic construct
GGTGLDTAI

SEQ ID NO: 42153 - protein, 9 aa, synthetic construct
GGTGLDTAV

SEQ ID NO: 42154 - protein, 9 aa, synthetic construct
GGTGLDTFA

SEQ ID NO: 42155 - protein, 9 aa, synthetic construct
GGTGLDTFV

SEQ ID NO: 42156 - protein, 9 aa, synthetic construct
GGTGLDTFY

SEQ ID NO: 42157 - protein, 9 aa, synthetic construct
GGTGLDTIE

SEQ ID NO: 42158 - protein, 9 aa, synthetic construct
GGTGLDTIR

SEQ ID NO: 42159 - protein, 9 aa, synthetic construct
GGTGLDTIS

SEQ ID NO: 42160 - protein, 9 aa, synthetic construct
GGTGLDTIW

SEQ ID NO: 42161 - protein, 9 aa, synthetic construct
GGTGLDTLD

SEQ ID NO: 42162 - protein, 9 aa, synthetic construct
GGTGLDTLE

SEQ ID NO: 42163 - protein, 9 aa, synthetic construct
GGTGLDTLS

SEQ ID NO: 42164 - protein, 9 aa, synthetic construct
GGTGLDTLW

SEQ ID NO: 42165 - protein, 9 aa, synthetic construct
GGTGLDTME

SEQ ID NO: 42166 - protein, 9 aa, synthetic construct
GGTGLDTML

SEQ ID NO: 42167 - protein, 9 aa, synthetic construct
GGTGLDTVR

SEQ ID NO: 42168 - protein, 9 aa, synthetic construct
GGTGLDTVV

SEQ ID NO: 42169 - protein, 9 aa, synthetic construct
GGTGLDVAV

SEQ ID NO: 42170 - protein, 9 aa, synthetic construct
GGTGLDVLI

SEQ ID NO: 42171 - protein, 9 aa, synthetic construct
GGTGLDVLV

SEQ ID NO: 42172 - protein, 9 aa, synthetic construct
GGTGLDVLY

SEQ ID NO: 42173 - protein, 9 aa, synthetic construct
GGTGLDYAD

SEQ ID NO: 42174 - protein, 9 aa, synthetic construct
GGTGLDYAS

SEQ ID NO: 42175 - protein, 9 aa, synthetic construct
GGTGLDYFI

SEQ ID NO: 42176 - protein, 9 aa, synthetic construct
GGTGLDYLN

SEQ ID NO: 42177 - protein, 9 aa, synthetic construct
GGTGLDYLT

SEQ ID NO: 42178 - protein, 9 aa, synthetic construct
GGTGLDYMD

SEQ ID NO: 42179 - protein, 9 aa, synthetic construct
GGTGMDEIM

SEQ ID NO: 42180 - protein, 9 aa, synthetic construct
GGTGLDTAD

SEQ ID NO: 42181 - protein, 9 aa, synthetic construct
GGTGLDSMI

SEQ ID NO: 42182 - protein, 9 aa, synthetic construct
GGTGLDSIN

SEQ ID NO: 42183 - protein, 9 aa, synthetic construct
GGTGLDLLV

SEQ ID NO: 42184 - protein, 9 aa, synthetic construct
GGTGLDFFT

SEQ ID NO: 42185 - protein, 9 aa, synthetic construct
GGTGLDIAD

SEQ ID NO: 42186 - protein, 9 aa, synthetic construct
GGTGLDIAI

SEQ ID NO: 42187 - protein, 9 aa, synthetic construct
GGTGLDIAS

SEQ ID NO: 42188 - protein, 9 aa, synthetic construct
GGTGLDIIG

SEQ ID NO: 42189 - protein, 9 aa, synthetic construct
GGTGLDILD

SEQ ID NO: 42190 - protein, 9 aa, synthetic construct
GGTGLDILI

SEQ ID NO: 42191 - protein, 9 aa, synthetic construct
GGTGLDILT

SEQ ID NO: 42192 - protein, 9 aa, synthetic construct
GGTGLDIVS

SEQ ID NO: 42193 - protein, 9 aa, synthetic construct
GGTGLDKLT

SEQ ID NO: 42194 - protein, 9 aa, synthetic construct
GGTGLDLFV

SEQ ID NO: 42195 - protein, 9 aa, synthetic construct
GGTGLDLIG

SEQ ID NO: 42196 - protein, 9 aa, synthetic construct
GGTGLDLLT

SEQ ID NO: 42197 - protein, 9 aa, synthetic construct
GGTGLDMLF

SEQ ID NO: 42198 - protein, 9 aa, synthetic construct
GGTGLDSAI

SEQ ID NO: 42199 - protein, 9 aa, synthetic construct
GGTGLDNYH

SEQ ID NO: 42200 - protein, 9 aa, synthetic construct
GGTGLDQIF

SEQ ID NO: 42201 - protein, 9 aa, synthetic construct
GGTGLDQLF

SEQ ID NO: 42202 - protein, 9 aa, synthetic construct
GGTGLDQLL

SEQ ID NO: 42203 - protein, 9 aa, synthetic construct
GGTGLDQLT

SEQ ID NO: 42204 - protein, 9 aa, synthetic construct
GGTGLDQLY

SEQ ID NO: 42205 - protein, 9 aa, synthetic construct
GGTGLDRIN

SEQ ID NO: 42206 - protein, 9 aa, synthetic construct
GGTGLDRIS

SEQ ID NO: 42207 - protein, 9 aa, synthetic construct
GGTGLDRLE

SEQ ID NO: 42208 - protein, 9 aa, synthetic construct
GGTGLDRLF

SEQ ID NO: 42209 - protein, 9 aa, synthetic construct
GGTGLDRLS

SEQ ID NO: 42210 - protein, 9 aa, synthetic construct
GGTGLDRLT

SEQ ID NO: 42211 - protein, 9 aa, synthetic construct
GGTGLDRMH

SEQ ID NO: 42212 - protein, 9 aa, synthetic construct
GGTGMDELR

SEQ ID NO: 42213 - protein, 9 aa, synthetic construct
GGTGMDILY

SEQ ID NO: 42214 - protein, 9 aa, synthetic construct
GGTGMDMVF

SEQ ID NO: 42215 - protein, 9 aa, synthetic construct
GGTGNDDYR

SEQ ID NO: 42216 - protein, 9 aa, synthetic construct
GGTGNDCMT

SEQ ID NO: 42217 - protein, 9 aa, synthetic construct
GGTGNDDAR

SEQ ID NO: 42218 - protein, 9 aa, synthetic construct
GGTGNDDAS

SEQ ID NO: 42219 - protein, 9 aa, synthetic construct
GGTGNDDFI

SEQ ID NO: 42220 - protein, 9 aa, synthetic construct
GGTGNDDIY

SEQ ID NO: 42221 - protein, 9 aa, synthetic construct
GGTGNDDLF

SEQ ID NO: 42222 - protein, 9 aa, synthetic construct
GGTGNDDLI

SEQ ID NO: 42223 - protein, 9 aa, synthetic construct
GGTGNDDLK

SEQ ID NO: 42224 - protein, 9 aa, synthetic construct
GGTGNDDLN

SEQ ID NO: 42225 - protein, 9 aa, synthetic construct
GGTGNDDLT

SEQ ID NO: 42226 - protein, 9 aa, synthetic construct
GGTGNDDMS

SEQ ID NO: 42227 - protein, 9 aa, synthetic construct
GGTGNDDMV

SEQ ID NO: 42228 - protein, 9 aa, synthetic construct
GGTGNDDVD

SEQ ID NO: 42229 - protein, 9 aa, synthetic construct
GGTGNDEFI

SEQ ID NO: 42230 - protein, 9 aa, synthetic construct
GGTGNDAYY

SEQ ID NO: 42231 - protein, 9 aa, synthetic construct
GGTGNDEFV

SEQ ID NO: 42232 - protein, 9 aa, synthetic construct
GGTGNDEIA

SEQ ID NO: 42233 - protein, 9 aa, synthetic construct
GGTGNDEIE

SEQ ID NO: 42234 - protein, 9 aa, synthetic construct
GGTGNDEIH

SEQ ID NO: 42235 - protein, 9 aa, synthetic construct
GGTGNDEIL

SEQ ID NO: 42236 - protein, 9 aa, synthetic construct
GGTGNDEIT

SEQ ID NO: 42237 - protein, 9 aa, synthetic construct
GGTGNDEIY

SEQ ID NO: 42238 - protein, 9 aa, synthetic construct
GGTGNDELA

SEQ ID NO: 42239 - protein, 9 aa, synthetic construct
GGTGNDELL

SEQ ID NO: 42240 - protein, 9 aa, synthetic construct
GGTGNDEME

SEQ ID NO: 42241 - protein, 9 aa, synthetic construct
GGTGNDEMF

SEQ ID NO: 42242 - protein, 9 aa, synthetic construct
GGTGNDEMI

SEQ ID NO: 42243 - protein, 9 aa, synthetic construct
GGTGNDEML

SEQ ID NO: 42244 - protein, 9 aa, synthetic construct
GGTGNDCLN

SEQ ID NO: 42245 - protein, 9 aa, synthetic construct
GGTGNDAYF

SEQ ID NO: 42246 - protein, 9 aa, synthetic construct
GGTGMDNVN

SEQ ID NO: 42247 - protein, 9 aa, synthetic construct
GGTGMDVMV

SEQ ID NO: 42248 - protein, 9 aa, synthetic construct
GGTGMDRIY

SEQ ID NO: 42249 - protein, 9 aa, synthetic construct
GGTGMDSLD

SEQ ID NO: 42250 - protein, 9 aa, synthetic construct
GGTGMDSLV

SEQ ID NO: 42251 - protein, 9 aa, synthetic construct
GGTGMDTAS

SEQ ID NO: 42252 - protein, 9 aa, synthetic construct
GGTGMDTFI

SEQ ID NO: 42253 - protein, 9 aa, synthetic construct
GGTGMDTLD

SEQ ID NO: 42254 - protein, 9 aa, synthetic construct
GGTGMDTLE

SEQ ID NO: 42255 - protein, 9 aa, synthetic construct
GGTGMDTLG

SEQ ID NO: 42256 - protein, 9 aa, synthetic construct
GGTGMDTLR

SEQ ID NO: 42257 - protein, 9 aa, synthetic construct
GGTGMDTLS

SEQ ID NO: 42258 - protein, 9 aa, synthetic construct
GGTGMDTVF

SEQ ID NO: 42259 - protein, 9 aa, synthetic construct
GGTGMDVLH

SEQ ID NO: 42260 - protein, 9 aa, synthetic construct
GGTGMDVLW

SEQ ID NO: 42261 - protein, 9 aa, synthetic construct
GGTGMDYAD

SEQ ID NO: 42262 - protein, 9 aa, synthetic construct
GGTGNDAYD

SEQ ID NO: 42263 - protein, 9 aa, synthetic construct
GGTGMDYVD

SEQ ID NO: 42264 - protein, 9 aa, synthetic construct
GGTGNDAFV

SEQ ID NO: 42265 - protein, 9 aa, synthetic construct
GGTGNDAFY

SEQ ID NO: 42266 - protein, 9 aa, synthetic construct
GGTGNDAIE

SEQ ID NO: 42267 - protein, 9 aa, synthetic construct
GGTGNDAIL

SEQ ID NO: 42268 - protein, 9 aa, synthetic construct
GGTGNDAIR

SEQ ID NO: 42269 - protein, 9 aa, synthetic construct
GGTGNDAIT

SEQ ID NO: 42270 - protein, 9 aa, synthetic construct
GGTGNDALE

SEQ ID NO: 42271 - protein, 9 aa, synthetic construct
GGTGNDALG

SEQ ID NO: 42272 - protein, 9 aa, synthetic construct
GGTGNDAMA

SEQ ID NO: 42273 - protein, 9 aa, synthetic construct
GGTGNDAMF

SEQ ID NO: 42274 - protein, 9 aa, synthetic construct
GGTGNDAMV

SEQ ID NO: 42275 - protein, 9 aa, synthetic construct
GGTGNDAVL

SEQ ID NO: 42276 - protein, 9 aa, synthetic construct
GGTGLDELY

SEQ ID NO: 42277 - protein, 9 aa, synthetic construct
GGTGLDDLY

SEQ ID NO: 42278 - protein, 9 aa, synthetic construct
GGTGIDSAY

SEQ ID NO: 42279 - protein, 9 aa, synthetic construct
GGTGLDDLS

SEQ ID NO: 42280 - protein, 9 aa, synthetic construct
GGTGKDAFN

SEQ ID NO: 42281 - protein, 9 aa, synthetic construct
GGTGKDALH

SEQ ID NO: 42282 - protein, 9 aa, synthetic construct
GGTGKDALN

SEQ ID NO: 42283 - protein, 9 aa, synthetic construct
GGTGKDALY

SEQ ID NO: 42284 - protein, 9 aa, synthetic construct
GGTGKDAVI

SEQ ID NO: 42285 - protein, 9 aa, synthetic construct
GGTGKDCFV

SEQ ID NO: 42286 - protein, 9 aa, synthetic construct
GGTGKDCIN

SEQ ID NO: 42287 - protein, 9 aa, synthetic construct
GGTGKDDIF

SEQ ID NO: 42288 - protein, 9 aa, synthetic construct
GGTGKDELY

SEQ ID NO: 42289 - protein, 9 aa, synthetic construct
GGTGKDFLV

SEQ ID NO: 42290 - protein, 9 aa, synthetic construct
GGTGKDGLT

SEQ ID NO: 42291 - protein, 9 aa, synthetic construct
GGTGKDHLA

SEQ ID NO: 42292 - protein, 9 aa, synthetic construct
GGTGKDHLK

SEQ ID NO: 42293 - protein, 9 aa, synthetic construct
GGTGKDIFK

SEQ ID NO: 42294 - protein, 9 aa, synthetic construct
GGTGKDIID

SEQ ID NO: 42295 - protein, 9 aa, synthetic construct
GGTGKDILD

SEQ ID NO: 42296 - protein, 9 aa, synthetic construct
GGTGKDILF

SEQ ID NO: 42297 - protein, 9 aa, synthetic construct
GGTGKDILG

SEQ ID NO: 42298 - protein, 9 aa, synthetic construct
GGTGKDILN

SEQ ID NO: 42299 - protein, 9 aa, synthetic construct
GGTGKDILS

SEQ ID NO: 42300 - protein, 9 aa, synthetic construct
GGTGKDILY

SEQ ID NO: 42301 - protein, 9 aa, synthetic construct
GGTGKDIMS

SEQ ID NO: 42302 - protein, 9 aa, synthetic construct
GGTGKDIVY

SEQ ID NO: 42303 - protein, 9 aa, synthetic construct
GGTGKDKFV

SEQ ID NO: 42304 - protein, 9 aa, synthetic construct
GGTGKDKIY

SEQ ID NO: 42305 - protein, 9 aa, synthetic construct
GGTGKDKLD

SEQ ID NO: 42306 - protein, 9 aa, synthetic construct
GGTGKDKLE

SEQ ID NO: 42307 - protein, 9 aa, synthetic construct
GGTGKDKVV

SEQ ID NO: 42308 - protein, 9 aa, synthetic construct
GGTGKDLAS

SEQ ID NO: 42309 - protein, 9 aa, synthetic construct
GGTGIDYLY

SEQ ID NO: 42310 - protein, 9 aa, synthetic construct
GGTGIDYLV

SEQ ID NO: 42311 - protein, 9 aa, synthetic construct
GGTGIDVMD

SEQ ID NO: 42312 - protein, 9 aa, synthetic construct
GGTGIDTIE

SEQ ID NO: 42313 - protein, 9 aa, synthetic construct
GGTGIDSFD

SEQ ID NO: 42314 - protein, 9 aa, synthetic construct
GGTGIDSIT

SEQ ID NO: 42315 - protein, 9 aa, synthetic construct
GGTGIDSLA

SEQ ID NO: 42316 - protein, 9 aa, synthetic construct
GGTGIDSLF

SEQ ID NO: 42317 - protein, 9 aa, synthetic construct
GGTGIDSLI

SEQ ID NO: 42318 - protein, 9 aa, synthetic construct
GGTGIDSLL

SEQ ID NO: 42319 - protein, 9 aa, synthetic construct
GGTGIDSMD

SEQ ID NO: 42320 - protein, 9 aa, synthetic construct
GGTGIDSML

SEQ ID NO: 42321 - protein, 9 aa, synthetic construct
GGTGIDSMS

SEQ ID NO: 42322 - protein, 9 aa, synthetic construct
GGTGIDSMV

SEQ ID NO: 42323 - protein, 9 aa, synthetic construct
GGTGIDSVL

SEQ ID NO: 42324 - protein, 9 aa, synthetic construct
GGTGIDTAL

SEQ ID NO: 42325 - protein, 9 aa, synthetic construct
GGTGIDTAQ

SEQ ID NO: 42326 - protein, 9 aa, synthetic construct
GGTGIDTIV

SEQ ID NO: 42327 - protein, 9 aa, synthetic construct
GGTGIDVMA

SEQ ID NO: 42328 - protein, 9 aa, synthetic construct
GGTGIDTLQ

SEQ ID NO: 42329 - protein, 9 aa, synthetic construct
GGTGIDTLV

SEQ ID NO: 42330 - protein, 9 aa, synthetic construct
GGTGIDTMA

SEQ ID NO: 42331 - protein, 9 aa, synthetic construct
GGTGIDTMM

SEQ ID NO: 42332 - protein, 9 aa, synthetic construct
GGTGIDTVL

SEQ ID NO: 42333 - protein, 9 aa, synthetic construct
GGTGIDTVT

SEQ ID NO: 42334 - protein, 9 aa, synthetic construct
GGTGIDTVY

SEQ ID NO: 42335 - protein, 9 aa, synthetic construct
GGTGIDTYD

SEQ ID NO: 42336 - protein, 9 aa, synthetic construct
GGTGIDVAD

SEQ ID NO: 42337 - protein, 9 aa, synthetic construct
GGTGIDVIR

SEQ ID NO: 42338 - protein, 9 aa, synthetic construct
GGTGIDVLL

SEQ ID NO: 42339 - protein, 9 aa, synthetic construct
GGTGIDVLN

SEQ ID NO: 42340 - protein, 9 aa, synthetic construct
GGTGIDVLY

SEQ ID NO: 42341 - protein, 9 aa, synthetic construct
GGTGKDLFI

SEQ ID NO: 42342 - protein, 9 aa, synthetic construct
GGTGKDLLF

SEQ ID NO: 42343 - protein, 9 aa, synthetic construct
GGTGKDLLG

SEQ ID NO: 42344 - protein, 9 aa, synthetic construct
GGTGKDVLI

SEQ ID NO: 42345 - protein, 9 aa, synthetic construct
GGTGKDTMF

SEQ ID NO: 42346 - protein, 9 aa, synthetic construct
GGTGKDTMH

SEQ ID NO: 42347 - protein, 9 aa, synthetic construct
GGTGKDTMK

SEQ ID NO: 42348 - protein, 9 aa, synthetic construct
GGTGKDTMR

SEQ ID NO: 42349 - protein, 9 aa, synthetic construct
GGTGKDTMV

SEQ ID NO: 42350 - protein, 9 aa, synthetic construct
GGTGKDTMY

SEQ ID NO: 42351 - protein, 9 aa, synthetic construct
GGTGKDTVL

SEQ ID NO: 42352 - protein, 9 aa, synthetic construct
GGTGKDTYV

SEQ ID NO: 42353 - protein, 9 aa, synthetic construct
GGTGKDVFA

SEQ ID NO: 42354 - protein, 9 aa, synthetic construct
GGTGKDVFM

SEQ ID NO: 42355 - protein, 9 aa, synthetic construct
GGTGKDVFR

SEQ ID NO: 42356 - protein, 9 aa, synthetic construct
GGTGKDVIT

SEQ ID NO: 42357 - protein, 9 aa, synthetic construct
GGTGKDVIV

SEQ ID NO: 42358 - protein, 9 aa, synthetic construct
GGTGKDVLK

SEQ ID NO: 42359 - protein, 9 aa, synthetic construct
GGTGKDTLG

SEQ ID NO: 42360 - protein, 9 aa, synthetic construct
GGTGKDVLN

SEQ ID NO: 42361 - protein, 9 aa, synthetic construct
GGTGKDVLQ

SEQ ID NO: 42362 - protein, 9 aa, synthetic construct
GGTGKDVLW

SEQ ID NO: 42363 - protein, 9 aa, synthetic construct
GGTGKDVME

SEQ ID NO: 42364 - protein, 9 aa, synthetic construct
GGTGKDVMI

SEQ ID NO: 42365 - protein, 9 aa, synthetic construct
GGTGKDVMR

SEQ ID NO: 42366 - protein, 9 aa, synthetic construct
GGTGKDWLD

SEQ ID NO: 42367 - protein, 9 aa, synthetic construct
GGTGKDYAS

SEQ ID NO: 42368 - protein, 9 aa, synthetic construct
GGTGKDYFV

SEQ ID NO: 42369 - protein, 9 aa, synthetic construct
GGTGKDYLF

SEQ ID NO: 42370 - protein, 9 aa, synthetic construct
GGTGLDAID

SEQ ID NO: 42371 - protein, 9 aa, synthetic construct
GGTGLDCVV

SEQ ID NO: 42372 - protein, 9 aa, synthetic construct
GGTGLDDFL

SEQ ID NO: 42373 - protein, 9 aa, synthetic construct
GGTGKDTLQ

SEQ ID NO: 42374 - protein, 9 aa, synthetic construct
GGTGKDTIY

SEQ ID NO: 42375 - protein, 9 aa, synthetic construct
GGTGKDLLT

SEQ ID NO: 42376 - protein, 9 aa, synthetic construct
GGTGKDRLL

SEQ ID NO: 42377 - protein, 9 aa, synthetic construct
GGTGKDLLY

SEQ ID NO: 42378 - protein, 9 aa, synthetic construct
GGTGKDLML

SEQ ID NO: 42379 - protein, 9 aa, synthetic construct
GGTGKDLMT

SEQ ID NO: 42380 - protein, 9 aa, synthetic construct
GGTGKDMFV

SEQ ID NO: 42381 - protein, 9 aa, synthetic construct
GGTGKDMLT

SEQ ID NO: 42382 - protein, 9 aa, synthetic construct
GGTGKDMLY

SEQ ID NO: 42383 - protein, 9 aa, synthetic construct
GGTGKDNFN

SEQ ID NO: 42384 - protein, 9 aa, synthetic construct
GGTGKDQLT

SEQ ID NO: 42385 - protein, 9 aa, synthetic construct
GGTGKDQMF

SEQ ID NO: 42386 - protein, 9 aa, synthetic construct
GGTGKDRFV

SEQ ID NO: 42387 - protein, 9 aa, synthetic construct
GGTGKDRIE

SEQ ID NO: 42388 - protein, 9 aa, synthetic construct
GGTGKDRIL

SEQ ID NO: 42389 - protein, 9 aa, synthetic construct
GGTGKDRIY

SEQ ID NO: 42390 - protein, 9 aa, synthetic construct
GGTGKDRMF

SEQ ID NO: 42391 - protein, 9 aa, synthetic construct
GGTGKDTIT

SEQ ID NO: 42392 - protein, 9 aa, synthetic construct
GGTGKDSFI

SEQ ID NO: 42393 - protein, 9 aa, synthetic construct
GGTGKDSIN

SEQ ID NO: 42394 - protein, 9 aa, synthetic construct
GGTGKDSIW

SEQ ID NO: 42395 - protein, 9 aa, synthetic construct
GGTGKDSLD

SEQ ID NO: 42396 - protein, 9 aa, synthetic construct
GGTGKDSLK

SEQ ID NO: 42397 - protein, 9 aa, synthetic construct
GGTGKDSLL

SEQ ID NO: 42398 - protein, 9 aa, synthetic construct
GGTGKDSMY

SEQ ID NO: 42399 - protein, 9 aa, synthetic construct
GGTGKDTAI

SEQ ID NO: 42400 - protein, 9 aa, synthetic construct
GGTGKDTAS

SEQ ID NO: 42401 - protein, 9 aa, synthetic construct
GGTGKDTAY

SEQ ID NO: 42402 - protein, 9 aa, synthetic construct
GGTGKDTFI

SEQ ID NO: 42403 - protein, 9 aa, synthetic construct
GGTGKDTID

SEQ ID NO: 42404 - protein, 9 aa, synthetic construct
GGTGKDTII

SEQ ID NO: 42405 - protein, 9 aa, synthetic construct
GGPGDDTMA

SEQ ID NO: 42406 - protein, 9 aa, synthetic construct
GGPGDDTIG

SEQ ID NO: 42407 - protein, 9 aa, synthetic construct
GGEGQDRMS

SEQ ID NO: 42408 - protein, 9 aa, synthetic construct
GGGGVDTLK

SEQ ID NO: 42409 - protein, 9 aa, synthetic construct
GGGGVDLLL

SEQ ID NO: 42410 - protein, 9 aa, synthetic construct
GGGGVDLLY

SEQ ID NO: 42411 - protein, 9 aa, synthetic construct
GGGGVDLVL

SEQ ID NO: 42412 - protein, 9 aa, synthetic construct
GGGGVDLVT

SEQ ID NO: 42413 - protein, 9 aa, synthetic construct
GGGGVDLVY

SEQ ID NO: 42414 - protein, 9 aa, synthetic construct
GGGGVDMLN

SEQ ID NO: 42415 - protein, 9 aa, synthetic construct
GGGGVDQFV

SEQ ID NO: 42416 - protein, 9 aa, synthetic construct
GGGGVDQLF

SEQ ID NO: 42417 - protein, 9 aa, synthetic construct
GGGGVDQLS

SEQ ID NO: 42418 - protein, 9 aa, synthetic construct
GGGGVDQLW

SEQ ID NO: 42419 - protein, 9 aa, synthetic construct
GGGGVDQMF

SEQ ID NO: 42420 - protein, 9 aa, synthetic construct
GGGGVDQMV

SEQ ID NO: 42421 - protein, 9 aa, synthetic construct
GGGGVDRAW

SEQ ID NO: 42422 - protein, 9 aa, synthetic construct
GGGGVDRFV

SEQ ID NO: 42423 - protein, 9 aa, synthetic construct
GGGGVDRIF

SEQ ID NO: 42424 - protein, 9 aa, synthetic construct
GGGGVDRIS

SEQ ID NO: 42425 - protein, 9 aa, synthetic construct
GGGGVDRYH

SEQ ID NO: 42426 - protein, 9 aa, synthetic construct
GGGGVDSID

SEQ ID NO: 42427 - protein, 9 aa, synthetic construct
GGGGVDSIR

SEQ ID NO: 42428 - protein, 9 aa, synthetic construct
GGGGVDSIS

SEQ ID NO: 42429 - protein, 9 aa, synthetic construct
GGGGVDSLV

SEQ ID NO: 42430 - protein, 9 aa, synthetic construct
GGGGVDSMS

SEQ ID NO: 42431 - protein, 9 aa, synthetic construct
GGGGVDSVY

SEQ ID NO: 42432 - protein, 9 aa, synthetic construct
GGGGVDTAA

SEQ ID NO: 42433 - protein, 9 aa, synthetic construct
GGGGVDTFC

SEQ ID NO: 42434 - protein, 9 aa, synthetic construct
GGGGVDTFL

SEQ ID NO: 42435 - protein, 9 aa, synthetic construct
GGGGVDTFN

SEQ ID NO: 42436 - protein, 9 aa, synthetic construct
GGGGVDTIA

SEQ ID NO: 42437 - protein, 9 aa, synthetic construct
GGGGVDTIE

SEQ ID NO: 42438 - protein, 9 aa, synthetic construct
GGGGVDLLD

SEQ ID NO: 42439 - protein, 9 aa, synthetic construct
GGGGVDLID

SEQ ID NO: 42440 - protein, 9 aa, synthetic construct
GGGGVDLAN

SEQ ID NO: 42441 - protein, 9 aa, synthetic construct
GGGGVDGAR

SEQ ID NO: 42442 - protein, 9 aa, synthetic construct
GGGGVDAFR

SEQ ID NO: 42443 - protein, 9 aa, synthetic construct
GGGGVDAFV

SEQ ID NO: 42444 - protein, 9 aa, synthetic construct
GGGGVDAID

SEQ ID NO: 42445 - protein, 9 aa, synthetic construct
GGGGVDAIH

SEQ ID NO: 42446 - protein, 9 aa, synthetic construct
GGGGVDALD

SEQ ID NO: 42447 - protein, 9 aa, synthetic construct
GGGGVDDLA

SEQ ID NO: 42448 - protein, 9 aa, synthetic construct
GGGGVDDLR

SEQ ID NO: 42449 - protein, 9 aa, synthetic construct
GGGGVDDLS

SEQ ID NO: 42450 - protein, 9 aa, synthetic construct
GGGGVDDVY

SEQ ID NO: 42451 - protein, 9 aa, synthetic construct
GGGGVDEIF

SEQ ID NO: 42452 - protein, 9 aa, synthetic construct
GGGGVDFID

SEQ ID NO: 42453 - protein, 9 aa, synthetic construct
GGGGVDFLL

SEQ ID NO: 42454 - protein, 9 aa, synthetic construct
GGGGVDFLT

SEQ ID NO: 42455 - protein, 9 aa, synthetic construct
GGGGVDHLI

SEQ ID NO: 42456 - protein, 9 aa, synthetic construct
GGGGVDKLH

SEQ ID NO: 42457 - protein, 9 aa, synthetic construct
GGGGVDHLS

SEQ ID NO: 42458 - protein, 9 aa, synthetic construct
GGGGVDIAD

SEQ ID NO: 42459 - protein, 9 aa, synthetic construct
GGGGVDIAV

SEQ ID NO: 42460 - protein, 9 aa, synthetic construct
GGGGVDIID

SEQ ID NO: 42461 - protein, 9 aa, synthetic construct
GGGGVDILI

SEQ ID NO: 42462 - protein, 9 aa, synthetic construct
GGGGVDIME

SEQ ID NO: 42463 - protein, 9 aa, synthetic construct
GGGGVDIMR

SEQ ID NO: 42464 - protein, 9 aa, synthetic construct
GGGGVDIVD

SEQ ID NO: 42465 - protein, 9 aa, synthetic construct
GGGGVDIVR

SEQ ID NO: 42466 - protein, 9 aa, synthetic construct
GGGGVDIVS

SEQ ID NO: 42467 - protein, 9 aa, synthetic construct
GGGGVDIYE

SEQ ID NO: 42468 - protein, 9 aa, synthetic construct
GGGGVDKFK

SEQ ID NO: 42469 - protein, 9 aa, synthetic construct
GGGGVDKLF

SEQ ID NO: 42470 - protein, 9 aa, synthetic construct
GGGGVDTLA

SEQ ID NO: 42471 - protein, 9 aa, synthetic construct
GGGGVDTLQ

SEQ ID NO: 42472 - protein, 9 aa, synthetic construct
GGGGYDVLI

SEQ ID NO: 42473 - protein, 9 aa, synthetic construct
GGGGVDTLR

SEQ ID NO: 42474 - protein, 9 aa, synthetic construct
GGGGYDLLE

SEQ ID NO: 42475 - protein, 9 aa, synthetic construct
GGGGYDLLI

SEQ ID NO: 42476 - protein, 9 aa, synthetic construct
GGGGYDLLM

SEQ ID NO: 42477 - protein, 9 aa, synthetic construct
GGGGYDLLR

SEQ ID NO: 42478 - protein, 9 aa, synthetic construct
GGGGYDLLV

SEQ ID NO: 42479 - protein, 9 aa, synthetic construct
GGGGYDLLY

SEQ ID NO: 42480 - protein, 9 aa, synthetic construct
GGGGYDLMY

SEQ ID NO: 42481 - protein, 9 aa, synthetic construct
GGGGYDLVT

SEQ ID NO: 42482 - protein, 9 aa, synthetic construct
GGGGYDMMQ

SEQ ID NO: 42483 - protein, 9 aa, synthetic construct
GGGGYDQLV

SEQ ID NO: 42484 - protein, 9 aa, synthetic construct
GGGGYDQVD

SEQ ID NO: 42485 - protein, 9 aa, synthetic construct
GGGGYDQVW

SEQ ID NO: 42486 - protein, 9 aa, synthetic construct
GGGGYDRLA

SEQ ID NO: 42487 - protein, 9 aa, synthetic construct
GGGGYDRLF

SEQ ID NO: 42488 - protein, 9 aa, synthetic construct
GGGGYDRLT

SEQ ID NO: 42489 - protein, 9 aa, synthetic construct
GGGGYDRMD

SEQ ID NO: 42490 - protein, 9 aa, synthetic construct
GGGGYDSLD

SEQ ID NO: 42491 - protein, 9 aa, synthetic construct
GGGGYDSLK

SEQ ID NO: 42492 - protein, 9 aa, synthetic construct
GGGGYDTAV

SEQ ID NO: 42493 - protein, 9 aa, synthetic construct
GGGGYDTIT

SEQ ID NO: 42494 - protein, 9 aa, synthetic construct
GGGGYDTLE

SEQ ID NO: 42495 - protein, 9 aa, synthetic construct
GGGGYDTLL

SEQ ID NO: 42496 - protein, 9 aa, synthetic construct
GGGGYDTLN

SEQ ID NO: 42497 - protein, 9 aa, synthetic construct
GGGGYDTLV

SEQ ID NO: 42498 - protein, 9 aa, synthetic construct
GGGGYDTLW

SEQ ID NO: 42499 - protein, 9 aa, synthetic construct
GGGGYDTVE

SEQ ID NO: 42500 - protein, 9 aa, synthetic construct
GGGGYDTYE

SEQ ID NO: 42501 - protein, 9 aa, synthetic construct
GGGGYDTYI

SEQ ID NO: 42502 - protein, 9 aa, synthetic construct
GGGGYDVAE

SEQ ID NO: 42503 - protein, 9 aa, synthetic construct
GGGGYDKLY

SEQ ID NO: 42504 - protein, 9 aa, synthetic construct
GGGGYDILL

SEQ ID NO: 42505 - protein, 9 aa, synthetic construct
GGGGYDILI

SEQ ID NO: 42506 - protein, 9 aa, synthetic construct
GGGGVDYLT

SEQ ID NO: 42507 - protein, 9 aa, synthetic construct
GGGGVDTMN

SEQ ID NO: 42508 - protein, 9 aa, synthetic construct
GGGGVDTMS

SEQ ID NO: 42509 - protein, 9 aa, synthetic construct
GGGGVDTMV

SEQ ID NO: 42510 - protein, 9 aa, synthetic construct
GGGGVDTVD

SEQ ID NO: 42511 - protein, 9 aa, synthetic construct
GGGGVDTVN

SEQ ID NO: 42512 - protein, 9 aa, synthetic construct
GGGGVDTVS

SEQ ID NO: 42513 - protein, 9 aa, synthetic construct
GGGGVDTYH

SEQ ID NO: 42514 - protein, 9 aa, synthetic construct
GGGGVDVFI

SEQ ID NO: 42515 - protein, 9 aa, synthetic construct
GGGGVDVLS

SEQ ID NO: 42516 - protein, 9 aa, synthetic construct
GGGGVDVMI

SEQ ID NO: 42517 - protein, 9 aa, synthetic construct
GGGGVDYFA

SEQ ID NO: 42518 - protein, 9 aa, synthetic construct
GGGGVDYFV

SEQ ID NO: 42519 - protein, 9 aa, synthetic construct
GGGGVDYLN

SEQ ID NO: 42520 - protein, 9 aa, synthetic construct
GGGGWDDLT

SEQ ID NO: 42521 - protein, 9 aa, synthetic construct
GGGGYDGLT

SEQ ID NO: 42522 - protein, 9 aa, synthetic construct
GGGGWDEFR

SEQ ID NO: 42523 - protein, 9 aa, synthetic construct
GGGGWDKLI

SEQ ID NO: 42524 - protein, 9 aa, synthetic construct
GGGGWDKLY

SEQ ID NO: 42525 - protein, 9 aa, synthetic construct
GGGGWDQLR

SEQ ID NO: 42526 - protein, 9 aa, synthetic construct
GGGGWDSLF

SEQ ID NO: 42527 - protein, 9 aa, synthetic construct
GGGGWDTLY

SEQ ID NO: 42528 - protein, 9 aa, synthetic construct
GGGGWDVIS

SEQ ID NO: 42529 - protein, 9 aa, synthetic construct
GGGGWDVLR

SEQ ID NO: 42530 - protein, 9 aa, synthetic construct
GGGGWDVLS

SEQ ID NO: 42531 - protein, 9 aa, synthetic construct
GGGGXDLIS

SEQ ID NO: 42532 - protein, 9 aa, synthetic construct
GGGGYDEIY

SEQ ID NO: 42533 - protein, 9 aa, synthetic construct
GGGGYDELL

SEQ ID NO: 42534 - protein, 9 aa, synthetic construct
GGGGYDELY

SEQ ID NO: 42535 - protein, 9 aa, synthetic construct
GGGGTDYVS

SEQ ID NO: 42536 - protein, 9 aa, synthetic construct
GGGGTDYLV

SEQ ID NO: 42537 - protein, 9 aa, synthetic construct
GGGGTDYLD

SEQ ID NO: 42538 - protein, 9 aa, synthetic construct
GGGGTDYFV

SEQ ID NO: 42539 - protein, 9 aa, synthetic construct
GGGGSDVIV

SEQ ID NO: 42540 - protein, 9 aa, synthetic construct
GGGGSDVLE

SEQ ID NO: 42541 - protein, 9 aa, synthetic construct
GGGGSDVLG

SEQ ID NO: 42542 - protein, 9 aa, synthetic construct
GGGGSDVLS

SEQ ID NO: 42543 - protein, 9 aa, synthetic construct
GGGGSDVMD

SEQ ID NO: 42544 - protein, 9 aa, synthetic construct
GGGGSDVMY

SEQ ID NO: 42545 - protein, 9 aa, synthetic construct
GGGGSDVYK

SEQ ID NO: 42546 - protein, 9 aa, synthetic construct
GGGGSDVYR

SEQ ID NO: 42547 - protein, 9 aa, synthetic construct
GGGGSDVYV

SEQ ID NO: 42548 - protein, 9 aa, synthetic construct
GGGGSDWAA

SEQ ID NO: 42549 - protein, 9 aa, synthetic construct
GGGGSDWAS

SEQ ID NO: 42550 - protein, 9 aa, synthetic construct
GGGGSDWIH

SEQ ID NO: 42551 - protein, 9 aa, synthetic construct
GGGGSDWLE

SEQ ID NO: 42552 - protein, 9 aa, synthetic construct
GGGGSDWLY

SEQ ID NO: 42553 - protein, 9 aa, synthetic construct
GGGGSDYLD

SEQ ID NO: 42554 - protein, 9 aa, synthetic construct
GGGGSDYLG

SEQ ID NO: 42555 - protein, 9 aa, synthetic construct
GGGGSDYLY

SEQ ID NO: 42556 - protein, 9 aa, synthetic construct
GGGGSDYMI

SEQ ID NO: 42557 - protein, 9 aa, synthetic construct
GGGGSDYMN

SEQ ID NO: 42558 - protein, 9 aa, synthetic construct
GGGGSDYMY

SEQ ID NO: 42559 - protein, 9 aa, synthetic construct
GGGGTDALF

SEQ ID NO: 42560 - protein, 9 aa, synthetic construct
GGGGTDALN

SEQ ID NO: 42561 - protein, 9 aa, synthetic construct
GGGGTDAVR

SEQ ID NO: 42562 - protein, 9 aa, synthetic construct
GGGGTDAVS

SEQ ID NO: 42563 - protein, 9 aa, synthetic construct
GGGGTDCIT

SEQ ID NO: 42564 - protein, 9 aa, synthetic construct
GGGGTDDLR

SEQ ID NO: 42565 - protein, 9 aa, synthetic construct
GGGGTDDLY

SEQ ID NO: 42566 - protein, 9 aa, synthetic construct
GGGGTDEMY

SEQ ID NO: 42567 - protein, 9 aa, synthetic construct
GGGGTDFAS

SEQ ID NO: 42568 - protein, 9 aa, synthetic construct
GGGGSDVIN

SEQ ID NO: 42569 - protein, 9 aa, synthetic construct
GGGGSDVIL

SEQ ID NO: 42570 - protein, 9 aa, synthetic construct
GGGGSDVFN

SEQ ID NO: 42571 - protein, 9 aa, synthetic construct
GGGGSDTMM

SEQ ID NO: 42572 - protein, 9 aa, synthetic construct
GGGGSDTAT

SEQ ID NO: 42573 - protein, 9 aa, synthetic construct
GGGGSDTAW

SEQ ID NO: 42574 - protein, 9 aa, synthetic construct
GGGGSDTFN

SEQ ID NO: 42575 - protein, 9 aa, synthetic construct
GGGGSDTFY

SEQ ID NO: 42576 - protein, 9 aa, synthetic construct
GGGGSDTIE

SEQ ID NO: 42577 - protein, 9 aa, synthetic construct
GGGGSDTIH

SEQ ID NO: 42578 - protein, 9 aa, synthetic construct
GGGGSDTIS

SEQ ID NO: 42579 - protein, 9 aa, synthetic construct
GGGGSDTIW

SEQ ID NO: 42580 - protein, 9 aa, synthetic construct
GGGGSDTLG

SEQ ID NO: 42581 - protein, 9 aa, synthetic construct
GGGGSDTLK

SEQ ID NO: 42582 - protein, 9 aa, synthetic construct
GGGGSDTLQ

SEQ ID NO: 42583 - protein, 9 aa, synthetic construct
GGGGSDTLW

SEQ ID NO: 42584 - protein, 9 aa, synthetic construct
GGGGSDTMD

SEQ ID NO: 42585 - protein, 9 aa, synthetic construct
GGGGSDTMR

SEQ ID NO: 42586 - protein, 9 aa, synthetic construct
GGGGSDVFK

SEQ ID NO: 42587 - protein, 9 aa, synthetic construct
GGGGSDTMY

SEQ ID NO: 42588 - protein, 9 aa, synthetic construct
GGGGSDTVA

SEQ ID NO: 42589 - protein, 9 aa, synthetic construct
GGGGSDTVD

SEQ ID NO: 42590 - protein, 9 aa, synthetic construct
GGGGSDTVH

SEQ ID NO: 42591 - protein, 9 aa, synthetic construct
GGGGSDTVI

SEQ ID NO: 42592 - protein, 9 aa, synthetic construct
GGGGSDTVY

SEQ ID NO: 42593 - protein, 9 aa, synthetic construct
GGGGSDTYF

SEQ ID NO: 42594 - protein, 9 aa, synthetic construct
GGGGSDTYQ

SEQ ID NO: 42595 - protein, 9 aa, synthetic construct
GGGGSDTYV

SEQ ID NO: 42596 - protein, 9 aa, synthetic construct
GGGGSDTYY

SEQ ID NO: 42597 - protein, 9 aa, synthetic construct
GGGGSDVAK

SEQ ID NO: 42598 - protein, 9 aa, synthetic construct
GGGGSDVAV

SEQ ID NO: 42599 - protein, 9 aa, synthetic construct
GGGGSDVFE

SEQ ID NO: 42600 - protein, 9 aa, synthetic construct
GGGGTDFFR

SEQ ID NO: 42601 - protein, 9 aa, synthetic construct
GGGGTDFLD

SEQ ID NO: 42602 - protein, 9 aa, synthetic construct
GGGGTDFLE

SEQ ID NO: 42603 - protein, 9 aa, synthetic construct
GGGGTDTLR

SEQ ID NO: 42604 - protein, 9 aa, synthetic construct
GGGGTDSLF

SEQ ID NO: 42605 - protein, 9 aa, synthetic construct
GGGGTDSLV

SEQ ID NO: 42606 - protein, 9 aa, synthetic construct
GGGGTDTAA

SEQ ID NO: 42607 - protein, 9 aa, synthetic construct
GGGGTDTAE

SEQ ID NO: 42608 - protein, 9 aa, synthetic construct
GGGGTDTAI

SEQ ID NO: 42609 - protein, 9 aa, synthetic construct
GGGGTDTAL

SEQ ID NO: 42610 - protein, 9 aa, synthetic construct
GGGGTDTFA

SEQ ID NO: 42611 - protein, 9 aa, synthetic construct
GGGGTDTFT

SEQ ID NO: 42612 - protein, 9 aa, synthetic construct
GGGGTDTIA

SEQ ID NO: 42613 - protein, 9 aa, synthetic construct
GGGGTDTIH

SEQ ID NO: 42614 - protein, 9 aa, synthetic construct
GGGGTDTII

SEQ ID NO: 42615 - protein, 9 aa, synthetic construct
GGGGTDTIY

SEQ ID NO: 42616 - protein, 9 aa, synthetic construct
GGGGTDTLF

SEQ ID NO: 42617 - protein, 9 aa, synthetic construct
GGGGTDTMT

SEQ ID NO: 42618 - protein, 9 aa, synthetic construct
GGGGTDRVD

SEQ ID NO: 42619 - protein, 9 aa, synthetic construct
GGGGTDTVY

SEQ ID NO: 42620 - protein, 9 aa, synthetic construct
GGGGTDVAV

SEQ ID NO: 42621 - protein, 9 aa, synthetic construct
GGGGTDVII

SEQ ID NO: 42622 - protein, 9 aa, synthetic construct
GGGGTDVIL

SEQ ID NO: 42623 - protein, 9 aa, synthetic construct
GGGGTDVLL

SEQ ID NO: 42624 - protein, 9 aa, synthetic construct
GGGGTDVLR

SEQ ID NO: 42625 - protein, 9 aa, synthetic construct
GGGGTDVLS

SEQ ID NO: 42626 - protein, 9 aa, synthetic construct
GGGGTDVLT

SEQ ID NO: 42627 - protein, 9 aa, synthetic construct
GGGGTDVLY

SEQ ID NO: 42628 - protein, 9 aa, synthetic construct
GGGGTDVYI

SEQ ID NO: 42629 - protein, 9 aa, synthetic construct
GGGGTDWLE

SEQ ID NO: 42630 - protein, 9 aa, synthetic construct
GGGGTDWLK

SEQ ID NO: 42631 - protein, 9 aa, synthetic construct
GGGGTDYAK

SEQ ID NO: 42632 - protein, 9 aa, synthetic construct
GGGGTDSIT

SEQ ID NO: 42633 - protein, 9 aa, synthetic construct
GGGGTDRLY

SEQ ID NO: 42634 - protein, 9 aa, synthetic construct
GGGGTDFLQ

SEQ ID NO: 42635 - protein, 9 aa, synthetic construct
GGGGTDLAN

SEQ ID NO: 42636 - protein, 9 aa, synthetic construct
GGGGTDFLT

SEQ ID NO: 42637 - protein, 9 aa, synthetic construct
GGGGTDHIY

SEQ ID NO: 42638 - protein, 9 aa, synthetic construct
GGGGTDHLI

SEQ ID NO: 42639 - protein, 9 aa, synthetic construct
GGGGTDIAV

SEQ ID NO: 42640 - protein, 9 aa, synthetic construct
GGGGTDIIY

SEQ ID NO: 42641 - protein, 9 aa, synthetic construct
GGGGTDILD

SEQ ID NO: 42642 - protein, 9 aa, synthetic construct
GGGGTDILK

SEQ ID NO: 42643 - protein, 9 aa, synthetic construct
GGGGTDILL

SEQ ID NO: 42644 - protein, 9 aa, synthetic construct
GGGGTDILY

SEQ ID NO: 42645 - protein, 9 aa, synthetic construct
GGGGTDKID

SEQ ID NO: 42646 - protein, 9 aa, synthetic construct
GGGGTDKIS

SEQ ID NO: 42647 - protein, 9 aa, synthetic construct
GGGGTDKLD

SEQ ID NO: 42648 - protein, 9 aa, synthetic construct
GGGGTDKLY

SEQ ID NO: 42649 - protein, 9 aa, synthetic construct
GGGGTDLAS

SEQ ID NO: 42650 - protein, 9 aa, synthetic construct
GGGGTDRLN

SEQ ID NO: 42651 - protein, 9 aa, synthetic construct
GGGGTDLFN

SEQ ID NO: 42652 - protein, 9 aa, synthetic construct
GGGGTDLIF

SEQ ID NO: 42653 - protein, 9 aa, synthetic construct
GGGGTDLLA

SEQ ID NO: 42654 - protein, 9 aa, synthetic construct
GGGGTDLLL

SEQ ID NO: 42655 - protein, 9 aa, synthetic construct
GGGGTDLLV

SEQ ID NO: 42656 - protein, 9 aa, synthetic construct
GGGGTDMLK

SEQ ID NO: 42657 - protein, 9 aa, synthetic construct
GGGGTDMLT

SEQ ID NO: 42658 - protein, 9 aa, synthetic construct
GGGGTDMLY

SEQ ID NO: 42659 - protein, 9 aa, synthetic construct
GGGGTDNLS

SEQ ID NO: 42660 - protein, 9 aa, synthetic construct
GGGGTDQYA

SEQ ID NO: 42661 - protein, 9 aa, synthetic construct
GGGGTDRAQ

SEQ ID NO: 42662 - protein, 9 aa, synthetic construct
GGGGTDRIE

SEQ ID NO: 42663 - protein, 9 aa, synthetic construct
GGGGTDRIY

SEQ ID NO: 42664 - protein, 9 aa, synthetic construct
GGGGYDVAQ

SEQ ID NO: 42665 - protein, 9 aa, synthetic construct
GGGGYDVLM

SEQ ID NO: 42666 - protein, 9 aa, synthetic construct
GGGGSDTAL

SEQ ID NO: 42667 - protein, 9 aa, synthetic construct
GGHGNDHLE

SEQ ID NO: 42668 - protein, 9 aa, synthetic construct
GGHGIDLLI

SEQ ID NO: 42669 - protein, 9 aa, synthetic construct
GGHGKDALF

SEQ ID NO: 42670 - protein, 9 aa, synthetic construct
GGHGKDFIY

SEQ ID NO: 42671 - protein, 9 aa, synthetic construct
GGHGKDKLT

SEQ ID NO: 42672 - protein, 9 aa, synthetic construct
GGHGKDRLW

SEQ ID NO: 42673 - protein, 9 aa, synthetic construct
GGHGKDSLF

SEQ ID NO: 42674 - protein, 9 aa, synthetic construct
GGHGKDTII

SEQ ID NO: 42675 - protein, 9 aa, synthetic construct
GGHGKDTLI

SEQ ID NO: 42676 - protein, 9 aa, synthetic construct
GGHGKDVLD

SEQ ID NO: 42677 - protein, 9 aa, synthetic construct
GGHGKDWLD

SEQ ID NO: 42678 - protein, 9 aa, synthetic construct
GGHGLDLLI

SEQ ID NO: 42679 - protein, 9 aa, synthetic construct
GGHGLDTIF

SEQ ID NO: 42680 - protein, 9 aa, synthetic construct
GGHGLDTIT

SEQ ID NO: 42681 - protein, 9 aa, synthetic construct
GGHGLDVIH

SEQ ID NO: 42682 - protein, 9 aa, synthetic construct
GGHGMDTLY

SEQ ID NO: 42683 - protein, 9 aa, synthetic construct
GGHGNDALH

SEQ ID NO: 42684 - protein, 9 aa, synthetic construct
GGHGNDALN

SEQ ID NO: 42685 - protein, 9 aa, synthetic construct
GGHGNDALR

SEQ ID NO: 42686 - protein, 9 aa, synthetic construct
GGHGNDALS

SEQ ID NO: 42687 - protein, 9 aa, synthetic construct
GGHGNDEIH

SEQ ID NO: 42688 - protein, 9 aa, synthetic construct
GGHGNDEIY

SEQ ID NO: 42689 - protein, 9 aa, synthetic construct
GGHGNDELM

SEQ ID NO: 42690 - protein, 9 aa, synthetic construct
GGHGNDELN

SEQ ID NO: 42691 - protein, 9 aa, synthetic construct
GGHGNDEMH

SEQ ID NO: 42692 - protein, 9 aa, synthetic construct
GGHGNDFIL

SEQ ID NO: 42693 - protein, 9 aa, synthetic construct
GGHGNDFIN

SEQ ID NO: 42694 - protein, 9 aa, synthetic construct
GGHGNDFLS

SEQ ID NO: 42695 - protein, 9 aa, synthetic construct
GGHGNDFLT

SEQ ID NO: 42696 - protein, 9 aa, synthetic construct
GGHGNDFMH

SEQ ID NO: 42697 - protein, 9 aa, synthetic construct
GGHGIDDLW

SEQ ID NO: 42698 - protein, 9 aa, synthetic construct
GGHGHDYLS

SEQ ID NO: 42699 - protein, 9 aa, synthetic construct
GGHGHDVMF

SEQ ID NO: 42700 - protein, 9 aa, synthetic construct
GGHGHDQVD

SEQ ID NO: 42701 - protein, 9 aa, synthetic construct
GGHGFDLLD

SEQ ID NO: 42702 - protein, 9 aa, synthetic construct
GGHGGDELR

SEQ ID NO: 42703 - protein, 9 aa, synthetic construct
GGHGGDIIL

SEQ ID NO: 42704 - protein, 9 aa, synthetic construct
GGHGGDILD

SEQ ID NO: 42705 - protein, 9 aa, synthetic construct
GGHGGDLIQ

SEQ ID NO: 42706 - protein, 9 aa, synthetic construct
GGHGGDLIY

SEQ ID NO: 42707 - protein, 9 aa, synthetic construct
GGHGGDQLG

SEQ ID NO: 42708 - protein, 9 aa, synthetic construct
GGHGGDRID

SEQ ID NO: 42709 - protein, 9 aa, synthetic construct
GGHGGDTYY

SEQ ID NO: 42710 - protein, 9 aa, synthetic construct
GGHGGDYMV

SEQ ID NO: 42711 - protein, 9 aa, synthetic construct
GGHGHDLLE

SEQ ID NO: 42712 - protein, 9 aa, synthetic construct
GGHGHDQFV

SEQ ID NO: 42713 - protein, 9 aa, synthetic construct
GGHGHDQMD

SEQ ID NO: 42714 - protein, 9 aa, synthetic construct
GGHGHDRLW

SEQ ID NO: 42715 - protein, 9 aa, synthetic construct
GGHGHDVLT

SEQ ID NO: 42716 - protein, 9 aa, synthetic construct
GGHGHDRLY

SEQ ID NO: 42717 - protein, 9 aa, synthetic construct
GGHGHDRMN

SEQ ID NO: 42718 - protein, 9 aa, synthetic construct
GGHGHDSLY

SEQ ID NO: 42719 - protein, 9 aa, synthetic construct
GGHGHDTFR

SEQ ID NO: 42720 - protein, 9 aa, synthetic construct
GGHGHDTLF

SEQ ID NO: 42721 - protein, 9 aa, synthetic construct
GGHGHDTLH

SEQ ID NO: 42722 - protein, 9 aa, synthetic construct
GGHGHDTLR

SEQ ID NO: 42723 - protein, 9 aa, synthetic construct
GGHGHDTLV

SEQ ID NO: 42724 - protein, 9 aa, synthetic construct
GGHGHDTLY

SEQ ID NO: 42725 - protein, 9 aa, synthetic construct
GGHGHDTVE

SEQ ID NO: 42726 - protein, 9 aa, synthetic construct
GGHGHDVFV

SEQ ID NO: 42727 - protein, 9 aa, synthetic construct
GGHGHDVIN

SEQ ID NO: 42728 - protein, 9 aa, synthetic construct
GGHGHDVLF

SEQ ID NO: 42729 - protein, 9 aa, synthetic construct
GGHGNDGLY

SEQ ID NO: 42730 - protein, 9 aa, synthetic construct
GGHGNDHLN

SEQ ID NO: 42731 - protein, 9 aa, synthetic construct
GGGGYDVMY

SEQ ID NO: 42732 - protein, 9 aa, synthetic construct
GGHGNDHLS

SEQ ID NO: 42733 - protein, 9 aa, synthetic construct
GGHGNDRLN

SEQ ID NO: 42734 - protein, 9 aa, synthetic construct
GGHGNDRVF

SEQ ID NO: 42735 - protein, 9 aa, synthetic construct
GGHGNDRYE

SEQ ID NO: 42736 - protein, 9 aa, synthetic construct
GGHGNDSIR

SEQ ID NO: 42737 - protein, 9 aa, synthetic construct
GGHGNDSIW

SEQ ID NO: 42738 - protein, 9 aa, synthetic construct
GGHGNDSLA

SEQ ID NO: 42739 - protein, 9 aa, synthetic construct
GGHGNDSLF

SEQ ID NO: 42740 - protein, 9 aa, synthetic construct
GGHGNDSLI

SEQ ID NO: 42741 - protein, 9 aa, synthetic construct
GGHGNDSLM

SEQ ID NO: 42742 - protein, 9 aa, synthetic construct
GGHGNDSLQ

SEQ ID NO: 42743 - protein, 9 aa, synthetic construct
GGHGNDSLR

SEQ ID NO: 42744 - protein, 9 aa, synthetic construct
GGHGNDTFI

SEQ ID NO: 42745 - protein, 9 aa, synthetic construct
GGHGNDTIE

SEQ ID NO: 42746 - protein, 9 aa, synthetic construct
GGHGNDTII

SEQ ID NO: 42747 - protein, 9 aa, synthetic construct
GGHGNDTIL

SEQ ID NO: 42748 - protein, 9 aa, synthetic construct
GGHGNDTIT

SEQ ID NO: 42749 - protein, 9 aa, synthetic construct
GGHGNDTIV

SEQ ID NO: 42750 - protein, 9 aa, synthetic construct
GGHGNDTLQ

SEQ ID NO: 42751 - protein, 9 aa, synthetic construct
GGHGNDTVH

SEQ ID NO: 42752 - protein, 9 aa, synthetic construct
GGHGNDTYF

SEQ ID NO: 42753 - protein, 9 aa, synthetic construct
GGHGNDTYL

SEQ ID NO: 42754 - protein, 9 aa, synthetic construct
GGHGNDVFF

SEQ ID NO: 42755 - protein, 9 aa, synthetic construct
GGHGNDVFV

SEQ ID NO: 42756 - protein, 9 aa, synthetic construct
GGHGNDVIA

SEQ ID NO: 42757 - protein, 9 aa, synthetic construct
GGHGNDVID

SEQ ID NO: 42758 - protein, 9 aa, synthetic construct
GGHGNDVIL

SEQ ID NO: 42759 - protein, 9 aa, synthetic construct
GGHGNDVIR

SEQ ID NO: 42760 - protein, 9 aa, synthetic construct
GGHGNDVIS

SEQ ID NO: 42761 - protein, 9 aa, synthetic construct
GGHGNDVLD

SEQ ID NO: 42762 - protein, 9 aa, synthetic construct
GGHGNDRLI

SEQ ID NO: 42763 - protein, 9 aa, synthetic construct
GGHGNDRLF

SEQ ID NO: 42764 - protein, 9 aa, synthetic construct
GGHGNDRLD

SEQ ID NO: 42765 - protein, 9 aa, synthetic construct
GGHGNDLVY

SEQ ID NO: 42766 - protein, 9 aa, synthetic construct
GGHGNDHLY

SEQ ID NO: 42767 - protein, 9 aa, synthetic construct
GGHGNDIFK

SEQ ID NO: 42768 - protein, 9 aa, synthetic construct
GGHGNDIIE

SEQ ID NO: 42769 - protein, 9 aa, synthetic construct
GGHGNDILE

SEQ ID NO: 42770 - protein, 9 aa, synthetic construct
GGHGNDILL

SEQ ID NO: 42771 - protein, 9 aa, synthetic construct
GGHGNDILS

SEQ ID NO: 42772 - protein, 9 aa, synthetic construct
GGHGNDILY

SEQ ID NO: 42773 - protein, 9 aa, synthetic construct
GGHGNDKLL

SEQ ID NO: 42774 - protein, 9 aa, synthetic construct
GGHGNDLID

SEQ ID NO: 42775 - protein, 9 aa, synthetic construct
GGHGNDLLS

SEQ ID NO: 42776 - protein, 9 aa, synthetic construct
GGHGNDLLV

SEQ ID NO: 42777 - protein, 9 aa, synthetic construct
GGHGNDLLY

SEQ ID NO: 42778 - protein, 9 aa, synthetic construct
GGHGNDLMA

SEQ ID NO: 42779 - protein, 9 aa, synthetic construct
GGHGNDLYN

SEQ ID NO: 42780 - protein, 9 aa, synthetic construct
GGHGNDRIE

SEQ ID NO: 42781 - protein, 9 aa, synthetic construct
GGHGNDMFR

SEQ ID NO: 42782 - protein, 9 aa, synthetic construct
GGHGNDMLT

SEQ ID NO: 42783 - protein, 9 aa, synthetic construct
GGHGNDMVI

SEQ ID NO: 42784 - protein, 9 aa, synthetic construct
GGHGNDMVK

SEQ ID NO: 42785 - protein, 9 aa, synthetic construct
GGHGNDNLW

SEQ ID NO: 42786 - protein, 9 aa, synthetic construct
GGHGNDNVL

SEQ ID NO: 42787 - protein, 9 aa, synthetic construct
GGHGNDQIF

SEQ ID NO: 42788 - protein, 9 aa, synthetic construct
GGHGNDQIG

SEQ ID NO: 42789 - protein, 9 aa, synthetic construct
GGHGNDQIN

SEQ ID NO: 42790 - protein, 9 aa, synthetic construct
GGHGNDQLA

SEQ ID NO: 42791 - protein, 9 aa, synthetic construct
GGHGNDQLE

SEQ ID NO: 42792 - protein, 9 aa, synthetic construct
GGHGNDQLI

SEQ ID NO: 42793 - protein, 9 aa, synthetic construct
GGHGNDRFH

SEQ ID NO: 42794 - protein, 9 aa, synthetic construct
GGHGFDILI

SEQ ID NO: 42795 - protein, 9 aa, synthetic construct
GGHGEDVLV

SEQ ID NO: 42796 - protein, 9 aa, synthetic construct
GGHGEDVLT

SEQ ID NO: 42797 - protein, 9 aa, synthetic construct
GGHGEDVLR

SEQ ID NO: 42798 - protein, 9 aa, synthetic construct
GGHGADTIE

SEQ ID NO: 42799 - protein, 9 aa, synthetic construct
GGHGADTIP

SEQ ID NO: 42800 - protein, 9 aa, synthetic construct
GGHGADTIT

SEQ ID NO: 42801 - protein, 9 aa, synthetic construct
GGHGADTLN

SEQ ID NO: 42802 - protein, 9 aa, synthetic construct
GGHGADTLV

SEQ ID NO: 42803 - protein, 9 aa, synthetic construct
GGHGADTYI

SEQ ID NO: 42804 - protein, 9 aa, synthetic construct
GGHGADVFC

SEQ ID NO: 42805 - protein, 9 aa, synthetic construct
GGHGADVFV

SEQ ID NO: 42806 - protein, 9 aa, synthetic construct
GGHGADVLK

SEQ ID NO: 42807 - protein, 9 aa, synthetic construct
GGHGADVLS

SEQ ID NO: 42808 - protein, 9 aa, synthetic construct
GGHGADVLV

SEQ ID NO: 42809 - protein, 9 aa, synthetic construct
GGHGADVVN

SEQ ID NO: 42810 - protein, 9 aa, synthetic construct
GGHGADYLS

SEQ ID NO: 42811 - protein, 9 aa, synthetic construct
GGHGDDAIT

SEQ ID NO: 42812 - protein, 9 aa, synthetic construct
GGHGDDALS

SEQ ID NO: 42813 - protein, 9 aa, synthetic construct
GGHGDDDLF

SEQ ID NO: 42814 - protein, 9 aa, synthetic construct
GGHGDDDLY

SEQ ID NO: 42815 - protein, 9 aa, synthetic construct
GGHGDDELL

SEQ ID NO: 42816 - protein, 9 aa, synthetic construct
GGHGDDFLN

SEQ ID NO: 42817 - protein, 9 aa, synthetic construct
GGHGDDGIA

SEQ ID NO: 42818 - protein, 9 aa, synthetic construct
GGHGDDHLA

SEQ ID NO: 42819 - protein, 9 aa, synthetic construct
GGHGDDHLD

SEQ ID NO: 42820 - protein, 9 aa, synthetic construct
GGHGDDHLS

SEQ ID NO: 42821 - protein, 9 aa, synthetic construct
GGHGDDIFV

SEQ ID NO: 42822 - protein, 9 aa, synthetic construct
GGHGDDILY

SEQ ID NO: 42823 - protein, 9 aa, synthetic construct
GGHGDDIMY

SEQ ID NO: 42824 - protein, 9 aa, synthetic construct
GGHGDDIVL

SEQ ID NO: 42825 - protein, 9 aa, synthetic construct
GGHGDDIYE

SEQ ID NO: 42826 - protein, 9 aa, synthetic construct
GGHGDDKIS

SEQ ID NO: 42827 - protein, 9 aa, synthetic construct
GGHGADSVE

SEQ ID NO: 42828 - protein, 9 aa, synthetic construct
GGHGADSLV

SEQ ID NO: 42829 - protein, 9 aa, synthetic construct
GGHGADSLS

SEQ ID NO: 42830 - protein, 9 aa, synthetic construct
GGHGADKLT

SEQ ID NO: 42831 - protein, 9 aa, synthetic construct
GGGGYDYLE

SEQ ID NO: 42832 - protein, 9 aa, synthetic construct
GGGGYDYLS

SEQ ID NO: 42833 - protein, 9 aa, synthetic construct
GGHGADDLH

SEQ ID NO: 42834 - protein, 9 aa, synthetic construct
GGHGADDLY

SEQ ID NO: 42835 - protein, 9 aa, synthetic construct
GGHGADEIL

SEQ ID NO: 42836 - protein, 9 aa, synthetic construct
GGHGADGLR

SEQ ID NO: 42837 - protein, 9 aa, synthetic construct
GGHGADHFL

SEQ ID NO: 42838 - protein, 9 aa, synthetic construct
GGHGADHFR

SEQ ID NO: 42839 - protein, 9 aa, synthetic construct
GGHGADHLF

SEQ ID NO: 42840 - protein, 9 aa, synthetic construct
GGHGADHLR

SEQ ID NO: 42841 - protein, 9 aa, synthetic construct
GGHGADILQ

SEQ ID NO: 42842 - protein, 9 aa, synthetic construct
GGHGADILR

SEQ ID NO: 42843 - protein, 9 aa, synthetic construct
GGHGADIMQ

SEQ ID NO: 42844 - protein, 9 aa, synthetic construct
GGHGADLIH

SEQ ID NO: 42845 - protein, 9 aa, synthetic construct
GGHGADSLL

SEQ ID NO: 42846 - protein, 9 aa, synthetic construct
GGHGADLLI

SEQ ID NO: 42847 - protein, 9 aa, synthetic construct
GGHGADLLR

SEQ ID NO: 42848 - protein, 9 aa, synthetic construct
GGHGADLLS

SEQ ID NO: 42849 - protein, 9 aa, synthetic construct
GGHGADMMV

SEQ ID NO: 42850 - protein, 9 aa, synthetic construct
GGHGADNID

SEQ ID NO: 42851 - protein, 9 aa, synthetic construct
GGHGADRFE

SEQ ID NO: 42852 - protein, 9 aa, synthetic construct
GGHGADRIV

SEQ ID NO: 42853 - protein, 9 aa, synthetic construct
GGHGADRMN

SEQ ID NO: 42854 - protein, 9 aa, synthetic construct
GGHGADRVN

SEQ ID NO: 42855 - protein, 9 aa, synthetic construct
GGHGADSIT

SEQ ID NO: 42856 - protein, 9 aa, synthetic construct
GGHGADSLD

SEQ ID NO: 42857 - protein, 9 aa, synthetic construct
GGHGADSLF

SEQ ID NO: 42858 - protein, 9 aa, synthetic construct
GGHGADSLI

SEQ ID NO: 42859 - protein, 9 aa, synthetic construct
GGHGDDKIY

SEQ ID NO: 42860 - protein, 9 aa, synthetic construct
GGHGDDKLS

SEQ ID NO: 42861 - protein, 9 aa, synthetic construct
GGHGDDLII

SEQ ID NO: 42862 - protein, 9 aa, synthetic construct
GGHGDDYLN

SEQ ID NO: 42863 - protein, 9 aa, synthetic construct
GGHGDDTVM

SEQ ID NO: 42864 - protein, 9 aa, synthetic construct
GGHGDDVAR

SEQ ID NO: 42865 - protein, 9 aa, synthetic construct
GGHGDDVIA

SEQ ID NO: 42866 - protein, 9 aa, synthetic construct
GGHGDDVIR

SEQ ID NO: 42867 - protein, 9 aa, synthetic construct
GGHGDDVLA

SEQ ID NO: 42868 - protein, 9 aa, synthetic construct
GGHGDDVLE

SEQ ID NO: 42869 - protein, 9 aa, synthetic construct
GGHGDDVLI

SEQ ID NO: 42870 - protein, 9 aa, synthetic construct
GGHGDDVLK

SEQ ID NO: 42871 - protein, 9 aa, synthetic construct
GGHGDDVLN

SEQ ID NO: 42872 - protein, 9 aa, synthetic construct
GGHGDDVLV

SEQ ID NO: 42873 - protein, 9 aa, synthetic construct
GGHGDDVLW

SEQ ID NO: 42874 - protein, 9 aa, synthetic construct
GGHGDDVVR

SEQ ID NO: 42875 - protein, 9 aa, synthetic construct
GGHGDDYLK

SEQ ID NO: 42876 - protein, 9 aa, synthetic construct
GGHGDDYLQ

SEQ ID NO: 42877 - protein, 9 aa, synthetic construct
GGHGDDTMY

SEQ ID NO: 42878 - protein, 9 aa, synthetic construct
GGHGDDYLS

SEQ ID NO: 42879 - protein, 9 aa, synthetic construct
GGHGDDYLY

SEQ ID NO: 42880 - protein, 9 aa, synthetic construct
GGHGEDALD

SEQ ID NO: 42881 - protein, 9 aa, synthetic construct
GGHGEDILA

SEQ ID NO: 42882 - protein, 9 aa, synthetic construct
GGHGEDILQ

SEQ ID NO: 42883 - protein, 9 aa, synthetic construct
GGHGEDNLS

SEQ ID NO: 42884 - protein, 9 aa, synthetic construct
GGHGEDRLL

SEQ ID NO: 42885 - protein, 9 aa, synthetic construct
GGHGEDSLV

SEQ ID NO: 42886 - protein, 9 aa, synthetic construct
GGHGEDTIL

SEQ ID NO: 42887 - protein, 9 aa, synthetic construct
GGHGEDTLI

SEQ ID NO: 42888 - protein, 9 aa, synthetic construct
GGHGEDTLL

SEQ ID NO: 42889 - protein, 9 aa, synthetic construct
GGHGEDTLR

SEQ ID NO: 42890 - protein, 9 aa, synthetic construct
GGHGEDVLH

SEQ ID NO: 42891 - protein, 9 aa, synthetic construct
GGHGDDTVH

SEQ ID NO: 42892 - protein, 9 aa, synthetic construct
GGHGDDTLT

SEQ ID NO: 42893 - protein, 9 aa, synthetic construct
GGHGDDLIS

SEQ ID NO: 42894 - protein, 9 aa, synthetic construct
GGHGDDRLS

SEQ ID NO: 42895 - protein, 9 aa, synthetic construct
GGHGDDLLD

SEQ ID NO: 42896 - protein, 9 aa, synthetic construct
GGHGDDLLN

SEQ ID NO: 42897 - protein, 9 aa, synthetic construct
GGHGDDLMV

SEQ ID NO: 42898 - protein, 9 aa, synthetic construct
GGHGDDLVL

SEQ ID NO: 42899 - protein, 9 aa, synthetic construct
GGHGDDMIH

SEQ ID NO: 42900 - protein, 9 aa, synthetic construct
GGHGDDMLN

SEQ ID NO: 42901 - protein, 9 aa, synthetic construct
GGHGDDNLD

SEQ ID NO: 42902 - protein, 9 aa, synthetic construct
GGHGDDNLN

SEQ ID NO: 42903 - protein, 9 aa, synthetic construct
GGHGDDQLF

SEQ ID NO: 42904 - protein, 9 aa, synthetic construct
GGHGDDRID

SEQ ID NO: 42905 - protein, 9 aa, synthetic construct
GGHGDDRIL

SEQ ID NO: 42906 - protein, 9 aa, synthetic construct
GGHGDDRLL

SEQ ID NO: 42907 - protein, 9 aa, synthetic construct
GGHGDDRLN

SEQ ID NO: 42908 - protein, 9 aa, synthetic construct
GGHGDDRMR

SEQ ID NO: 42909 - protein, 9 aa, synthetic construct
GGHGDDTLM

SEQ ID NO: 42910 - protein, 9 aa, synthetic construct
GGHGDDRMY

SEQ ID NO: 42911 - protein, 9 aa, synthetic construct
GGHGDDRVT

SEQ ID NO: 42912 - protein, 9 aa, synthetic construct
GGHGDDSID

SEQ ID NO: 42913 - protein, 9 aa, synthetic construct
GGHGDDSIF

SEQ ID NO: 42914 - protein, 9 aa, synthetic construct
GGHGDDSLK

SEQ ID NO: 42915 - protein, 9 aa, synthetic construct
GGHGDDSLR

SEQ ID NO: 42916 - protein, 9 aa, synthetic construct
GGHGDDSLS

SEQ ID NO: 42917 - protein, 9 aa, synthetic construct
GGHGDDSVF

SEQ ID NO: 42918 - protein, 9 aa, synthetic construct
GGHGDDTFV

SEQ ID NO: 42919 - protein, 9 aa, synthetic construct
GGHGDDTIF

SEQ ID NO: 42920 - protein, 9 aa, synthetic construct
GGHGDDTLE

SEQ ID NO: 42921 - protein, 9 aa, synthetic construct
GGHGDDTLG

SEQ ID NO: 42922 - protein, 9 aa, synthetic construct
GGHGDDTLH

SEQ ID NO: 42923 - protein, 9 aa, synthetic construct
GGGGSDTAM

SEQ ID NO: 42924 - protein, 9 aa, synthetic construct
GGGGSDTAI

SEQ ID NO: 42925 - protein, 9 aa, synthetic construct
GGKGDDCLA

SEQ ID NO: 42926 - protein, 9 aa, synthetic construct
GGGGNDVFH

SEQ ID NO: 42927 - protein, 9 aa, synthetic construct
GGGGNDSAI

SEQ ID NO: 42928 - protein, 9 aa, synthetic construct
GGGGNDSAS

SEQ ID NO: 42929 - protein, 9 aa, synthetic construct
GGGGNDSAY

SEQ ID NO: 42930 - protein, 9 aa, synthetic construct
GGGGNDSFD

SEQ ID NO: 42931 - protein, 9 aa, synthetic construct
GGGGNDSIH

SEQ ID NO: 42932 - protein, 9 aa, synthetic construct
GGGGNDSIV

SEQ ID NO: 42933 - protein, 9 aa, synthetic construct
GGGGNDSLH

SEQ ID NO: 42934 - protein, 9 aa, synthetic construct
GGGGNDSLM

SEQ ID NO: 42935 - protein, 9 aa, synthetic construct
GGGGNDSMA

SEQ ID NO: 42936 - protein, 9 aa, synthetic construct
GGGGNDSMI

SEQ ID NO: 42937 - protein, 9 aa, synthetic construct
GGGGNDSML

SEQ ID NO: 42938 - protein, 9 aa, synthetic construct
GGGGNDSMS

SEQ ID NO: 42939 - protein, 9 aa, synthetic construct
GGGGNDSVL

SEQ ID NO: 42940 - protein, 9 aa, synthetic construct
GGGGNDSYS

SEQ ID NO: 42941 - protein, 9 aa, synthetic construct
GGGGNDSYV

SEQ ID NO: 42942 - protein, 9 aa, synthetic construct
GGGGNDTAE

SEQ ID NO: 42943 - protein, 9 aa, synthetic construct
GGGGNDTAI

SEQ ID NO: 42944 - protein, 9 aa, synthetic construct
GGGGNDTAQ

SEQ ID NO: 42945 - protein, 9 aa, synthetic construct
GGGGNDTAY

SEQ ID NO: 42946 - protein, 9 aa, synthetic construct
GGGGNDTFE

SEQ ID NO: 42947 - protein, 9 aa, synthetic construct
GGGGNDTFN

SEQ ID NO: 42948 - protein, 9 aa, synthetic construct
GGGGNDTIP

SEQ ID NO: 42949 - protein, 9 aa, synthetic construct
GGGGNDTMA

SEQ ID NO: 42950 - protein, 9 aa, synthetic construct
GGGGNDTVF

SEQ ID NO: 42951 - protein, 9 aa, synthetic construct
GGGGNDTYT

SEQ ID NO: 42952 - protein, 9 aa, synthetic construct
GGGGNDVAD

SEQ ID NO: 42953 - protein, 9 aa, synthetic construct
GGGGNDVAI

SEQ ID NO: 42954 - protein, 9 aa, synthetic construct
GGGGNDVAL

SEQ ID NO: 42955 - protein, 9 aa, synthetic construct
GGGGNDVFD

SEQ ID NO: 42956 - protein, 9 aa, synthetic construct
GGGGNDSAD

SEQ ID NO: 42957 - protein, 9 aa, synthetic construct
GGGGNDRYI

SEQ ID NO: 42958 - protein, 9 aa, synthetic construct
GGGGNDRYA

SEQ ID NO: 42959 - protein, 9 aa, synthetic construct
GGGGNDQMY

SEQ ID NO: 42960 - protein, 9 aa, synthetic construct
GGGGNDNVN

SEQ ID NO: 42961 - protein, 9 aa, synthetic construct
GGGGNDNVT

SEQ ID NO: 42962 - protein, 9 aa, synthetic construct
GGGGNDNVY

SEQ ID NO: 42963 - protein, 9 aa, synthetic construct
GGGGNDNYI

SEQ ID NO: 42964 - protein, 9 aa, synthetic construct
GGGGNDPLN

SEQ ID NO: 42965 - protein, 9 aa, synthetic construct
GGGGNDQFA

SEQ ID NO: 42966 - protein, 9 aa, synthetic construct
GGGGNDQFT

SEQ ID NO: 42967 - protein, 9 aa, synthetic construct
GGGGNDQIL

SEQ ID NO: 42968 - protein, 9 aa, synthetic construct
GGGGNDQIN

SEQ ID NO: 42969 - protein, 9 aa, synthetic construct
GGGGNDQIT

SEQ ID NO: 42970 - protein, 9 aa, synthetic construct
GGGGNDQLD

SEQ ID NO: 42971 - protein, 9 aa, synthetic construct
GGGGNDQLE

SEQ ID NO: 42972 - protein, 9 aa, synthetic construct
GGGGNDQLI

SEQ ID NO: 42973 - protein, 9 aa, synthetic construct
GGGGNDQVF

SEQ ID NO: 42974 - protein, 9 aa, synthetic construct
GGGGNDRVW

SEQ ID NO: 42975 - protein, 9 aa, synthetic construct
GGGGNDQVS

SEQ ID NO: 42976 - protein, 9 aa, synthetic construct
GGGGNDRAM

SEQ ID NO: 42977 - protein, 9 aa, synthetic construct
GGGGNDRFF

SEQ ID NO: 42978 - protein, 9 aa, synthetic construct
GGGGNDRFH

SEQ ID NO: 42979 - protein, 9 aa, synthetic construct
GGGGNDRFT

SEQ ID NO: 42980 - protein, 9 aa, synthetic construct
GGGGNDRFV

SEQ ID NO: 42981 - protein, 9 aa, synthetic construct
GGGGNDRIA

SEQ ID NO: 42982 - protein, 9 aa, synthetic construct
GGGGNDRIH

SEQ ID NO: 42983 - protein, 9 aa, synthetic construct
GGGGNDRIT

SEQ ID NO: 42984 - protein, 9 aa, synthetic construct
GGGGNDRIV

SEQ ID NO: 42985 - protein, 9 aa, synthetic construct
GGGGNDRME

SEQ ID NO: 42986 - protein, 9 aa, synthetic construct
GGGGNDRMN

SEQ ID NO: 42987 - protein, 9 aa, synthetic construct
GGGGNDRVN

SEQ ID NO: 42988 - protein, 9 aa, synthetic construct
GGGGNDVFF

SEQ ID NO: 42989 - protein, 9 aa, synthetic construct
GGGGNDVFR

SEQ ID NO: 42990 - protein, 9 aa, synthetic construct
GGGGQDLLY

SEQ ID NO: 42991 - protein, 9 aa, synthetic construct
GGGGNDVFT

SEQ ID NO: 42992 - protein, 9 aa, synthetic construct
GGGGPDMLY

SEQ ID NO: 42993 - protein, 9 aa, synthetic construct
GGGGPDNLD

SEQ ID NO: 42994 - protein, 9 aa, synthetic construct
GGGGPDRLF

SEQ ID NO: 42995 - protein, 9 aa, synthetic construct
GGGGPDRLQ

SEQ ID NO: 42996 - protein, 9 aa, synthetic construct
GGGGPDRLR

SEQ ID NO: 42997 - protein, 9 aa, synthetic construct
GGGGPDSLS

SEQ ID NO: 42998 - protein, 9 aa, synthetic construct
GGGGPDTFF

SEQ ID NO: 42999 - protein, 9 aa, synthetic construct
GGGGPDTIV

SEQ ID NO: 43000 - protein, 9 aa, synthetic construct
GGGGPDTIY

SEQ ID NO: 43001 - protein, 9 aa, synthetic construct
GGGGPDTLI

SEQ ID NO: 43002 - protein, 9 aa, synthetic construct
GGGGPDTLY

SEQ ID NO: 43003 - protein, 9 aa, synthetic construct
GGGGPDTMH

SEQ ID NO: 43004 - protein, 9 aa, synthetic construct
GGGGPDVLI

SEQ ID NO: 43005 - protein, 9 aa, synthetic construct
GGGGQDALA

SEQ ID NO: 43006 - protein, 9 aa, synthetic construct
GGGGQDDLT

SEQ ID NO: 43007 - protein, 9 aa, synthetic construct
GGGGQDDMT

SEQ ID NO: 43008 - protein, 9 aa, synthetic construct
GGGGQDELQ

SEQ ID NO: 43009 - protein, 9 aa, synthetic construct
GGGGQDFAE

SEQ ID NO: 43010 - protein, 9 aa, synthetic construct
GGGGQDFFA

SEQ ID NO: 43011 - protein, 9 aa, synthetic construct
GGGGQDHFD

SEQ ID NO: 43012 - protein, 9 aa, synthetic construct
GGGGQDIFV

SEQ ID NO: 43013 - protein, 9 aa, synthetic construct
GGGGQDIIA

SEQ ID NO: 43014 - protein, 9 aa, synthetic construct
GGGGQDIII

SEQ ID NO: 43015 - protein, 9 aa, synthetic construct
GGGGQDILK

SEQ ID NO: 43016 - protein, 9 aa, synthetic construct
GGGGQDILL

SEQ ID NO: 43017 - protein, 9 aa, synthetic construct
GGGGQDLFR

SEQ ID NO: 43018 - protein, 9 aa, synthetic construct
GGGGQDLID

SEQ ID NO: 43019 - protein, 9 aa, synthetic construct
GGGGQDLIN

SEQ ID NO: 43020 - protein, 9 aa, synthetic construct
GGGGQDLLD

SEQ ID NO: 43021 - protein, 9 aa, synthetic construct
GGGGPDLLV

SEQ ID NO: 43022 - protein, 9 aa, synthetic construct
GGGGPDLLS

SEQ ID NO: 43023 - protein, 9 aa, synthetic construct
GGGGPDLIH

SEQ ID NO: 43024 - protein, 9 aa, synthetic construct
GGGGNDWLF

SEQ ID NO: 43025 - protein, 9 aa, synthetic construct
GGGGNDVIH

SEQ ID NO: 43026 - protein, 9 aa, synthetic construct
GGGGNDVIM

SEQ ID NO: 43027 - protein, 9 aa, synthetic construct
GGGGNDVIW

SEQ ID NO: 43028 - protein, 9 aa, synthetic construct
GGGGNDVMN

SEQ ID NO: 43029 - protein, 9 aa, synthetic construct
GGGGNDVMR

SEQ ID NO: 43030 - protein, 9 aa, synthetic construct
GGGGNDVMV

SEQ ID NO: 43031 - protein, 9 aa, synthetic construct
GGGGNDVVS

SEQ ID NO: 43032 - protein, 9 aa, synthetic construct
GGGGNDVVW

SEQ ID NO: 43033 - protein, 9 aa, synthetic construct
GGGGNDVYI

SEQ ID NO: 43034 - protein, 9 aa, synthetic construct
GGGGNDVYL

SEQ ID NO: 43035 - protein, 9 aa, synthetic construct
GGGGNDVYR

SEQ ID NO: 43036 - protein, 9 aa, synthetic construct
GGGGNDWFH

SEQ ID NO: 43037 - protein, 9 aa, synthetic construct
GGGGNDWIN

SEQ ID NO: 43038 - protein, 9 aa, synthetic construct
GGGGNDWMK

SEQ ID NO: 43039 - protein, 9 aa, synthetic construct
GGGGPDFLD

SEQ ID NO: 43040 - protein, 9 aa, synthetic construct
GGGGNDWMS

SEQ ID NO: 43041 - protein, 9 aa, synthetic construct
GGGGNDWMV

SEQ ID NO: 43042 - protein, 9 aa, synthetic construct
GGGGNDWVY

SEQ ID NO: 43043 - protein, 9 aa, synthetic construct
GGGGNDYAD

SEQ ID NO: 43044 - protein, 9 aa, synthetic construct
GGGGNDYIF

SEQ ID NO: 43045 - protein, 9 aa, synthetic construct
GGGGNDYIW

SEQ ID NO: 43046 - protein, 9 aa, synthetic construct
GGGGNDYLM

SEQ ID NO: 43047 - protein, 9 aa, synthetic construct
GGGGNDYLR

SEQ ID NO: 43048 - protein, 9 aa, synthetic construct
GGGGNDYMK

SEQ ID NO: 43049 - protein, 9 aa, synthetic construct
GGGGNDYVM

SEQ ID NO: 43050 - protein, 9 aa, synthetic construct
GGGGPDALN

SEQ ID NO: 43051 - protein, 9 aa, synthetic construct
GGGGPDALR

SEQ ID NO: 43052 - protein, 9 aa, synthetic construct
GGGGPDELS

SEQ ID NO: 43053 - protein, 9 aa, synthetic construct
GGGGNDNMV

SEQ ID NO: 43054 - protein, 9 aa, synthetic construct
GGGGNDNMT

SEQ ID NO: 43055 - protein, 9 aa, synthetic construct
GGGGNDNMG

SEQ ID NO: 43056 - protein, 9 aa, synthetic construct
GGGGNDNLV

SEQ ID NO: 43057 - protein, 9 aa, synthetic construct
GGGGNDFLK

SEQ ID NO: 43058 - protein, 9 aa, synthetic construct
GGGGNDFLV

SEQ ID NO: 43059 - protein, 9 aa, synthetic construct
GGGGNDFML

SEQ ID NO: 43060 - protein, 9 aa, synthetic construct
GGGGNDFMR

SEQ ID NO: 43061 - protein, 9 aa, synthetic construct
GGGGNDFVV

SEQ ID NO: 43062 - protein, 9 aa, synthetic construct
GGGGNDFYV

SEQ ID NO: 43063 - protein, 9 aa, synthetic construct
GGGGNDGFD

SEQ ID NO: 43064 - protein, 9 aa, synthetic construct
GGGGNDGIA

SEQ ID NO: 43065 - protein, 9 aa, synthetic construct
GGGGNDGID

SEQ ID NO: 43066 - protein, 9 aa, synthetic construct
GGGGNDGIR

SEQ ID NO: 43067 - protein, 9 aa, synthetic construct
GGGGNDGLF

SEQ ID NO: 43068 - protein, 9 aa, synthetic construct
GGGGNDGLT

SEQ ID NO: 43069 - protein, 9 aa, synthetic construct
GGGGNDGMV

SEQ ID NO: 43070 - protein, 9 aa, synthetic construct
GGGGNDGVA

SEQ ID NO: 43071 - protein, 9 aa, synthetic construct
GGGGNDGVS

SEQ ID NO: 43072 - protein, 9 aa, synthetic construct
GGGGNDGVW

SEQ ID NO: 43073 - protein, 9 aa, synthetic construct
GGGGNDHAF

SEQ ID NO: 43074 - protein, 9 aa, synthetic construct
GGGGNDHAS

SEQ ID NO: 43075 - protein, 9 aa, synthetic construct
GGGGNDHAT

SEQ ID NO: 43076 - protein, 9 aa, synthetic construct
GGGGNDHFK

SEQ ID NO: 43077 - protein, 9 aa, synthetic construct
GGGGNDHIH

SEQ ID NO: 43078 - protein, 9 aa, synthetic construct
GGGGNDHIL

SEQ ID NO: 43079 - protein, 9 aa, synthetic construct
GGGGNDHIV

SEQ ID NO: 43080 - protein, 9 aa, synthetic construct
GGGGNDHLN

SEQ ID NO: 43081 - protein, 9 aa, synthetic construct
GGGGNDHLQ

SEQ ID NO: 43082 - protein, 9 aa, synthetic construct
GGGGNDHLR

SEQ ID NO: 43083 - protein, 9 aa, synthetic construct
GGGGNDHLT

SEQ ID NO: 43084 - protein, 9 aa, synthetic construct
GGGGNDHLW

SEQ ID NO: 43085 - protein, 9 aa, synthetic construct
GGGGNDHMS

SEQ ID NO: 43086 - protein, 9 aa, synthetic construct
GGGGNDFLI

SEQ ID NO: 43087 - protein, 9 aa, synthetic construct
GGGGNDFLH

SEQ ID NO: 43088 - protein, 9 aa, synthetic construct
GGGGNDFIY

SEQ ID NO: 43089 - protein, 9 aa, synthetic construct
GGGGNDEFR

SEQ ID NO: 43090 - protein, 9 aa, synthetic construct
GGGGNDAYD

SEQ ID NO: 43091 - protein, 9 aa, synthetic construct
GGGGNDAYV

SEQ ID NO: 43092 - protein, 9 aa, synthetic construct
GGGGNDCIV

SEQ ID NO: 43093 - protein, 9 aa, synthetic construct
GGGGNDDIS

SEQ ID NO: 43094 - protein, 9 aa, synthetic construct
GGGGNDDIY

SEQ ID NO: 43095 - protein, 9 aa, synthetic construct
GGGGNDDLF

SEQ ID NO: 43096 - protein, 9 aa, synthetic construct
GGGGNDDLI

SEQ ID NO: 43097 - protein, 9 aa, synthetic construct
GGGGNDDLK

SEQ ID NO: 43098 - protein, 9 aa, synthetic construct
GGGGNDDLL

SEQ ID NO: 43099 - protein, 9 aa, synthetic construct
GGGGNDDLQ

SEQ ID NO: 43100 - protein, 9 aa, synthetic construct
GGGGNDDML

SEQ ID NO: 43101 - protein, 9 aa, synthetic construct
GGGGNDDVD

SEQ ID NO: 43102 - protein, 9 aa, synthetic construct
GGGGNDEFD

SEQ ID NO: 43103 - protein, 9 aa, synthetic construct
GGGGNDEII

SEQ ID NO: 43104 - protein, 9 aa, synthetic construct
GGGGNDFIQ

SEQ ID NO: 43105 - protein, 9 aa, synthetic construct
GGGGNDEIT

SEQ ID NO: 43106 - protein, 9 aa, synthetic construct
GGGGNDEIY

SEQ ID NO: 43107 - protein, 9 aa, synthetic construct
GGGGNDELG

SEQ ID NO: 43108 - protein, 9 aa, synthetic construct
GGGGNDELT

SEQ ID NO: 43109 - protein, 9 aa, synthetic construct
GGGGNDELV

SEQ ID NO: 43110 - protein, 9 aa, synthetic construct
GGGGNDELW

SEQ ID NO: 43111 - protein, 9 aa, synthetic construct
GGGGNDEMF

SEQ ID NO: 43112 - protein, 9 aa, synthetic construct
GGGGNDEMS

SEQ ID NO: 43113 - protein, 9 aa, synthetic construct
GGGGNDEVI

SEQ ID NO: 43114 - protein, 9 aa, synthetic construct
GGGGNDEVN

SEQ ID NO: 43115 - protein, 9 aa, synthetic construct
GGGGNDFAD

SEQ ID NO: 43116 - protein, 9 aa, synthetic construct
GGGGNDFIF

SEQ ID NO: 43117 - protein, 9 aa, synthetic construct
GGGGNDFIH

SEQ ID NO: 43118 - protein, 9 aa, synthetic construct
GGGGNDIAD

SEQ ID NO: 43119 - protein, 9 aa, synthetic construct
GGGGNDIFI

SEQ ID NO: 43120 - protein, 9 aa, synthetic construct
GGGGNDIIL

SEQ ID NO: 43121 - protein, 9 aa, synthetic construct
GGGGNDLYV

SEQ ID NO: 43122 - protein, 9 aa, synthetic construct
GGGGNDLMD

SEQ ID NO: 43123 - protein, 9 aa, synthetic construct
GGGGNDLME

SEQ ID NO: 43124 - protein, 9 aa, synthetic construct
GGGGNDLMI

SEQ ID NO: 43125 - protein, 9 aa, synthetic construct
GGGGNDLML

SEQ ID NO: 43126 - protein, 9 aa, synthetic construct
GGGGNDLMN

SEQ ID NO: 43127 - protein, 9 aa, synthetic construct
GGGGNDLMW

SEQ ID NO: 43128 - protein, 9 aa, synthetic construct
GGGGNDLVF

SEQ ID NO: 43129 - protein, 9 aa, synthetic construct
GGGGNDLVQ

SEQ ID NO: 43130 - protein, 9 aa, synthetic construct
GGGGNDLVR

SEQ ID NO: 43131 - protein, 9 aa, synthetic construct
GGGGNDLVT

SEQ ID NO: 43132 - protein, 9 aa, synthetic construct
GGGGNDLYI

SEQ ID NO: 43133 - protein, 9 aa, synthetic construct
GGGGNDLYK

SEQ ID NO: 43134 - protein, 9 aa, synthetic construct
GGGGNDLYR

SEQ ID NO: 43135 - protein, 9 aa, synthetic construct
GGGGNDMFV

SEQ ID NO: 43136 - protein, 9 aa, synthetic construct
GGGGNDLIT

SEQ ID NO: 43137 - protein, 9 aa, synthetic construct
GGGGNDMID

SEQ ID NO: 43138 - protein, 9 aa, synthetic construct
GGGGNDMII

SEQ ID NO: 43139 - protein, 9 aa, synthetic construct
GGGGNDMLG

SEQ ID NO: 43140 - protein, 9 aa, synthetic construct
GGGGNDMLM

SEQ ID NO: 43141 - protein, 9 aa, synthetic construct
GGGGNDMLV

SEQ ID NO: 43142 - protein, 9 aa, synthetic construct
GGGGNDMLW

SEQ ID NO: 43143 - protein, 9 aa, synthetic construct
GGGGNDMMI

SEQ ID NO: 43144 - protein, 9 aa, synthetic construct
GGGGNDMVT

SEQ ID NO: 43145 - protein, 9 aa, synthetic construct
GGGGNDNIF

SEQ ID NO: 43146 - protein, 9 aa, synthetic construct
GGGGNDNIQ

SEQ ID NO: 43147 - protein, 9 aa, synthetic construct
GGGGNDNIV

SEQ ID NO: 43148 - protein, 9 aa, synthetic construct
GGGGNDNIW

SEQ ID NO: 43149 - protein, 9 aa, synthetic construct
GGGGNDNLL

SEQ ID NO: 43150 - protein, 9 aa, synthetic construct
GGGGNDLLC

SEQ ID NO: 43151 - protein, 9 aa, synthetic construct
GGGGNDLIH

SEQ ID NO: 43152 - protein, 9 aa, synthetic construct
GGGGNDIIQ

SEQ ID NO: 43153 - protein, 9 aa, synthetic construct
GGGGNDKAF

SEQ ID NO: 43154 - protein, 9 aa, synthetic construct
GGGGNDILG

SEQ ID NO: 43155 - protein, 9 aa, synthetic construct
GGGGNDILK

SEQ ID NO: 43156 - protein, 9 aa, synthetic construct
GGGGNDILW

SEQ ID NO: 43157 - protein, 9 aa, synthetic construct
GGGGNDIVA

SEQ ID NO: 43158 - protein, 9 aa, synthetic construct
GGGGNDIVD

SEQ ID NO: 43159 - protein, 9 aa, synthetic construct
GGGGNDIVI

SEQ ID NO: 43160 - protein, 9 aa, synthetic construct
GGGGNDIVL

SEQ ID NO: 43161 - protein, 9 aa, synthetic construct
GGGGNDIVN

SEQ ID NO: 43162 - protein, 9 aa, synthetic construct
GGGGNDIVT

SEQ ID NO: 43163 - protein, 9 aa, synthetic construct
GGGGNDIVV

SEQ ID NO: 43164 - protein, 9 aa, synthetic construct
GGGGNDIYA

SEQ ID NO: 43165 - protein, 9 aa, synthetic construct
GGGGNDIYT

SEQ ID NO: 43166 - protein, 9 aa, synthetic construct
GGGGNDIYW

SEQ ID NO: 43167 - protein, 9 aa, synthetic construct
GGGGNDKFF

SEQ ID NO: 43168 - protein, 9 aa, synthetic construct
GGGGNDLFR

SEQ ID NO: 43169 - protein, 9 aa, synthetic construct
GGGGNDKFV

SEQ ID NO: 43170 - protein, 9 aa, synthetic construct
GGGGNDKID

SEQ ID NO: 43171 - protein, 9 aa, synthetic construct
GGGGNDKIG

SEQ ID NO: 43172 - protein, 9 aa, synthetic construct
GGGGNDKIV

SEQ ID NO: 43173 - protein, 9 aa, synthetic construct
GGGGNDKIY

SEQ ID NO: 43174 - protein, 9 aa, synthetic construct
GGGGNDKLH

SEQ ID NO: 43175 - protein, 9 aa, synthetic construct
GGGGNDKMS

SEQ ID NO: 43176 - protein, 9 aa, synthetic construct
GGGGNDKVY

SEQ ID NO: 43177 - protein, 9 aa, synthetic construct
GGGGNDLAS

SEQ ID NO: 43178 - protein, 9 aa, synthetic construct
GGGGNDLAY

SEQ ID NO: 43179 - protein, 9 aa, synthetic construct
GGGGNDLFA

SEQ ID NO: 43180 - protein, 9 aa, synthetic construct
GGGGNDLFN

SEQ ID NO: 43181 - protein, 9 aa, synthetic construct
GGGGNDLFQ

SEQ ID NO: 43182 - protein, 9 aa, synthetic construct
GGGGQDLLN

SEQ ID NO: 43183 - protein, 9 aa, synthetic construct
GGGGQDLMK

SEQ ID NO: 43184 - protein, 9 aa, synthetic construct
GGGGSDSMN

SEQ ID NO: 43185 - protein, 9 aa, synthetic construct
GGGGSDIFY

SEQ ID NO: 43186 - protein, 9 aa, synthetic construct
GGGGSDAML

SEQ ID NO: 43187 - protein, 9 aa, synthetic construct
GGGGSDAMS

SEQ ID NO: 43188 - protein, 9 aa, synthetic construct
GGGGSDAVI

SEQ ID NO: 43189 - protein, 9 aa, synthetic construct
GGGGSDAYY

SEQ ID NO: 43190 - protein, 9 aa, synthetic construct
GGGGSDDAN

SEQ ID NO: 43191 - protein, 9 aa, synthetic construct
GGGGSDDFG

SEQ ID NO: 43192 - protein, 9 aa, synthetic construct
GGGGSDDFV

SEQ ID NO: 43193 - protein, 9 aa, synthetic construct
GGGGSDDLF

SEQ ID NO: 43194 - protein, 9 aa, synthetic construct
GGGGSDDLR

SEQ ID NO: 43195 - protein, 9 aa, synthetic construct
GGGGSDDLV

SEQ ID NO: 43196 - protein, 9 aa, synthetic construct
GGGGSDDML

SEQ ID NO: 43197 - protein, 9 aa, synthetic construct
GGGGSDDVG

SEQ ID NO: 43198 - protein, 9 aa, synthetic construct
GGGGSDEFI

SEQ ID NO: 43199 - protein, 9 aa, synthetic construct
GGGGSDEIW

SEQ ID NO: 43200 - protein, 9 aa, synthetic construct
GGGGSDELD

SEQ ID NO: 43201 - protein, 9 aa, synthetic construct
GGGGSDELQ

SEQ ID NO: 43202 - protein, 9 aa, synthetic construct
GGGGSDELY

SEQ ID NO: 43203 - protein, 9 aa, synthetic construct
GGGGSDEMR

SEQ ID NO: 43204 - protein, 9 aa, synthetic construct
GGGGSDFIF

SEQ ID NO: 43205 - protein, 9 aa, synthetic construct
GGGGSDFIT

SEQ ID NO: 43206 - protein, 9 aa, synthetic construct
GGGGSDFLH

SEQ ID NO: 43207 - protein, 9 aa, synthetic construct
GGGGSDFLM

SEQ ID NO: 43208 - protein, 9 aa, synthetic construct
GGGGSDGLW

SEQ ID NO: 43209 - protein, 9 aa, synthetic construct
GGGGSDHLE

SEQ ID NO: 43210 - protein, 9 aa, synthetic construct
GGGGSDHLI

SEQ ID NO: 43211 - protein, 9 aa, synthetic construct
GGGGSDHLS

SEQ ID NO: 43212 - protein, 9 aa, synthetic construct
GGGGSDHLT

SEQ ID NO: 43213 - protein, 9 aa, synthetic construct
GGGGSDIFC

SEQ ID NO: 43214 - protein, 9 aa, synthetic construct
GGGGSDIFD

SEQ ID NO: 43215 - protein, 9 aa, synthetic construct
GGGGSDALV

SEQ ID NO: 43216 - protein, 9 aa, synthetic construct
GGGGSDALD

SEQ ID NO: 43217 - protein, 9 aa, synthetic construct
GGGGSDAIS

SEQ ID NO: 43218 - protein, 9 aa, synthetic construct
GGGGRDVIR

SEQ ID NO: 43219 - protein, 9 aa, synthetic construct
GGGGRDTLN

SEQ ID NO: 43220 - protein, 9 aa, synthetic construct
GGGGRDTLQ

SEQ ID NO: 43221 - protein, 9 aa, synthetic construct
GGGGRDTMI

SEQ ID NO: 43222 - protein, 9 aa, synthetic construct
GGGGRDTMR

SEQ ID NO: 43223 - protein, 9 aa, synthetic construct
GGGGRDTMS

SEQ ID NO: 43224 - protein, 9 aa, synthetic construct
GGGGRDTVN

SEQ ID NO: 43225 - protein, 9 aa, synthetic construct
GGGGRDTVY

SEQ ID NO: 43226 - protein, 9 aa, synthetic construct
GGGGRDVAH

SEQ ID NO: 43227 - protein, 9 aa, synthetic construct
GGGGRDVAQ

SEQ ID NO: 43228 - protein, 9 aa, synthetic construct
GGGGRDVFN

SEQ ID NO: 43229 - protein, 9 aa, synthetic construct
GGGGRDVIA

SEQ ID NO: 43230 - protein, 9 aa, synthetic construct
GGGGRDVIF

SEQ ID NO: 43231 - protein, 9 aa, synthetic construct
GGGGRDVIK

SEQ ID NO: 43232 - protein, 9 aa, synthetic construct
GGGGRDVIV

SEQ ID NO: 43233 - protein, 9 aa, synthetic construct
GGGGSDAID

SEQ ID NO: 43234 - protein, 9 aa, synthetic construct
GGGGRDVMA

SEQ ID NO: 43235 - protein, 9 aa, synthetic construct
GGGGRDVMR

SEQ ID NO: 43236 - protein, 9 aa, synthetic construct
GGGGRDVVY

SEQ ID NO: 43237 - protein, 9 aa, synthetic construct
GGGGRDVYS

SEQ ID NO: 43238 - protein, 9 aa, synthetic construct
GGGGRDWLT

SEQ ID NO: 43239 - protein, 9 aa, synthetic construct
GGGGRDWLY

SEQ ID NO: 43240 - protein, 9 aa, synthetic construct
GGGGRDYIL

SEQ ID NO: 43241 - protein, 9 aa, synthetic construct
GGGGRDYIS

SEQ ID NO: 43242 - protein, 9 aa, synthetic construct
GGGGRDYLF

SEQ ID NO: 43243 - protein, 9 aa, synthetic construct
GGGGRDYLN

SEQ ID NO: 43244 - protein, 9 aa, synthetic construct
GGGGSDAFC

SEQ ID NO: 43245 - protein, 9 aa, synthetic construct
GGGGSDAFG

SEQ ID NO: 43246 - protein, 9 aa, synthetic construct
GGGGSDAFV

SEQ ID NO: 43247 - protein, 9 aa, synthetic construct
GGGGSDIFT

SEQ ID NO: 43248 - protein, 9 aa, synthetic construct
GGGGSDIID

SEQ ID NO: 43249 - protein, 9 aa, synthetic construct
GGGGQDLVR

SEQ ID NO: 43250 - protein, 9 aa, synthetic construct
GGGGSDIIE

SEQ ID NO: 43251 - protein, 9 aa, synthetic construct
GGGGSDQLR

SEQ ID NO: 43252 - protein, 9 aa, synthetic construct
GGGGSDQLT

SEQ ID NO: 43253 - protein, 9 aa, synthetic construct
GGGGSDQLV

SEQ ID NO: 43254 - protein, 9 aa, synthetic construct
GGGGSDQLY

SEQ ID NO: 43255 - protein, 9 aa, synthetic construct
GGGGSDRIE

SEQ ID NO: 43256 - protein, 9 aa, synthetic construct
GGGGSDRIF

SEQ ID NO: 43257 - protein, 9 aa, synthetic construct
GGGGSDRII

SEQ ID NO: 43258 - protein, 9 aa, synthetic construct
GGGGSDRIS

SEQ ID NO: 43259 - protein, 9 aa, synthetic construct
GGGGSDRLK

SEQ ID NO: 43260 - protein, 9 aa, synthetic construct
GGGGSDRLL

SEQ ID NO: 43261 - protein, 9 aa, synthetic construct
GGGGSDRMA

SEQ ID NO: 43262 - protein, 9 aa, synthetic construct
GGGGSDRME

SEQ ID NO: 43263 - protein, 9 aa, synthetic construct
GGGGSDRMI

SEQ ID NO: 43264 - protein, 9 aa, synthetic construct
GGGGSDRMT

SEQ ID NO: 43265 - protein, 9 aa, synthetic construct
GGGGSDRVG

SEQ ID NO: 43266 - protein, 9 aa, synthetic construct
GGGGSDRVY

SEQ ID NO: 43267 - protein, 9 aa, synthetic construct
GGGGSDRYV

SEQ ID NO: 43268 - protein, 9 aa, synthetic construct
GGGGSDSFI

SEQ ID NO: 43269 - protein, 9 aa, synthetic construct
GGGGSDSFV

SEQ ID NO: 43270 - protein, 9 aa, synthetic construct
GGGGSDSID

SEQ ID NO: 43271 - protein, 9 aa, synthetic construct
GGGGSDSII

SEQ ID NO: 43272 - protein, 9 aa, synthetic construct
GGGGSDSIP

SEQ ID NO: 43273 - protein, 9 aa, synthetic construct
GGGGSDSLA

SEQ ID NO: 43274 - protein, 9 aa, synthetic construct
GGGGSDSLE

SEQ ID NO: 43275 - protein, 9 aa, synthetic construct
GGGGSDSLF

SEQ ID NO: 43276 - protein, 9 aa, synthetic construct
GGGGSDSLI

SEQ ID NO: 43277 - protein, 9 aa, synthetic construct
GGGGSDSLK

SEQ ID NO: 43278 - protein, 9 aa, synthetic construct
GGGGSDSLV

SEQ ID NO: 43279 - protein, 9 aa, synthetic construct
GGGGSDSLW

SEQ ID NO: 43280 - protein, 9 aa, synthetic construct
GGGGSDQLI

SEQ ID NO: 43281 - protein, 9 aa, synthetic construct
GGGGSDQLG

SEQ ID NO: 43282 - protein, 9 aa, synthetic construct
GGGGSDQIT

SEQ ID NO: 43283 - protein, 9 aa, synthetic construct
GGGGSDKLT

SEQ ID NO: 43284 - protein, 9 aa, synthetic construct
GGGGSDIIQ

SEQ ID NO: 43285 - protein, 9 aa, synthetic construct
GGGGSDIIS

SEQ ID NO: 43286 - protein, 9 aa, synthetic construct
GGGGSDIIW

SEQ ID NO: 43287 - protein, 9 aa, synthetic construct
GGGGSDILE

SEQ ID NO: 43288 - protein, 9 aa, synthetic construct
GGGGSDILV

SEQ ID NO: 43289 - protein, 9 aa, synthetic construct
GGGGSDILW

SEQ ID NO: 43290 - protein, 9 aa, synthetic construct
GGGGSDIMT

SEQ ID NO: 43291 - protein, 9 aa, synthetic construct
GGGGSDIVA

SEQ ID NO: 43292 - protein, 9 aa, synthetic construct
GGGGSDIVL

SEQ ID NO: 43293 - protein, 9 aa, synthetic construct
GGGGSDIVT

SEQ ID NO: 43294 - protein, 9 aa, synthetic construct
GGGGSDKIF

SEQ ID NO: 43295 - protein, 9 aa, synthetic construct
GGGGSDKIS

SEQ ID NO: 43296 - protein, 9 aa, synthetic construct
GGGGSDKLC

SEQ ID NO: 43297 - protein, 9 aa, synthetic construct
GGGGSDLFV

SEQ ID NO: 43298 - protein, 9 aa, synthetic construct
GGGGSDQFI

SEQ ID NO: 43299 - protein, 9 aa, synthetic construct
GGGGSDLIW

SEQ ID NO: 43300 - protein, 9 aa, synthetic construct
GGGGSDLMA

SEQ ID NO: 43301 - protein, 9 aa, synthetic construct
GGGGSDLMD

SEQ ID NO: 43302 - protein, 9 aa, synthetic construct
GGGGSDLMS

SEQ ID NO: 43303 - protein, 9 aa, synthetic construct
GGGGSDLVE

SEQ ID NO: 43304 - protein, 9 aa, synthetic construct
GGGGSDLVH

SEQ ID NO: 43305 - protein, 9 aa, synthetic construct
GGGGSDLVL

SEQ ID NO: 43306 - protein, 9 aa, synthetic construct
GGGGSDMLN

SEQ ID NO: 43307 - protein, 9 aa, synthetic construct
GGGGSDMLV

SEQ ID NO: 43308 - protein, 9 aa, synthetic construct
GGGGSDMMD

SEQ ID NO: 43309 - protein, 9 aa, synthetic construct
GGGGSDNFD

SEQ ID NO: 43310 - protein, 9 aa, synthetic construct
GGGGSDNFH

SEQ ID NO: 43311 - protein, 9 aa, synthetic construct
GGGGSDNLQ

SEQ ID NO: 43312 - protein, 9 aa, synthetic construct
GGGGRDTLH

SEQ ID NO: 43313 - protein, 9 aa, synthetic construct
GGGGRDTIN

SEQ ID NO: 43314 - protein, 9 aa, synthetic construct
GGGGRDTIL

SEQ ID NO: 43315 - protein, 9 aa, synthetic construct
GGGGRDTIK

SEQ ID NO: 43316 - protein, 9 aa, synthetic construct
GGGGQDTVI

SEQ ID NO: 43317 - protein, 9 aa, synthetic construct
GGGGQDTVR

SEQ ID NO: 43318 - protein, 9 aa, synthetic construct
GGGGQDVFI

SEQ ID NO: 43319 - protein, 9 aa, synthetic construct
GGGGQDVLK

SEQ ID NO: 43320 - protein, 9 aa, synthetic construct
GGGGQDVLL

SEQ ID NO: 43321 - protein, 9 aa, synthetic construct
GGGGQDYLL

SEQ ID NO: 43322 - protein, 9 aa, synthetic construct
GGGGQDYMN

SEQ ID NO: 43323 - protein, 9 aa, synthetic construct
GGGGRDAFV

SEQ ID NO: 43324 - protein, 9 aa, synthetic construct
GGGGRDAID

SEQ ID NO: 43325 - protein, 9 aa, synthetic construct
GGGGRDAIR

SEQ ID NO: 43326 - protein, 9 aa, synthetic construct
GGGGRDALD

SEQ ID NO: 43327 - protein, 9 aa, synthetic construct
GGGGRDALN

SEQ ID NO: 43328 - protein, 9 aa, synthetic construct
GGGGRDALR

SEQ ID NO: 43329 - protein, 9 aa, synthetic construct
GGGGRDAVS

SEQ ID NO: 43330 - protein, 9 aa, synthetic construct
GGGGRDDFL

SEQ ID NO: 43331 - protein, 9 aa, synthetic construct
GGGGRDDMI

SEQ ID NO: 43332 - protein, 9 aa, synthetic construct
GGGGRDDMV

SEQ ID NO: 43333 - protein, 9 aa, synthetic construct
GGGGRDEFH

SEQ ID NO: 43334 - protein, 9 aa, synthetic construct
GGGGRDEIF

SEQ ID NO: 43335 - protein, 9 aa, synthetic construct
GGGGRDEIR

SEQ ID NO: 43336 - protein, 9 aa, synthetic construct
GGGGRDELS

SEQ ID NO: 43337 - protein, 9 aa, synthetic construct
GGGGRDELV

SEQ ID NO: 43338 - protein, 9 aa, synthetic construct
GGGGRDFLF

SEQ ID NO: 43339 - protein, 9 aa, synthetic construct
GGGGRDFLM

SEQ ID NO: 43340 - protein, 9 aa, synthetic construct
GGGGRDFLQ

SEQ ID NO: 43341 - protein, 9 aa, synthetic construct
GGGGRDFLS

SEQ ID NO: 43342 - protein, 9 aa, synthetic construct
GGGGRDFMT

SEQ ID NO: 43343 - protein, 9 aa, synthetic construct
GGGGRDHFV

SEQ ID NO: 43344 - protein, 9 aa, synthetic construct
GGGGRDHLD

SEQ ID NO: 43345 - protein, 9 aa, synthetic construct
GGGGQDTMQ

SEQ ID NO: 43346 - protein, 9 aa, synthetic construct
GGGGQDTMH

SEQ ID NO: 43347 - protein, 9 aa, synthetic construct
GGGGQDTMF

SEQ ID NO: 43348 - protein, 9 aa, synthetic construct
GGGGQDSLW

SEQ ID NO: 43349 - protein, 9 aa, synthetic construct
GGGGQDQIS

SEQ ID NO: 43350 - protein, 9 aa, synthetic construct
GGGGQDQLD

SEQ ID NO: 43351 - protein, 9 aa, synthetic construct
GGGGQDQLL

SEQ ID NO: 43352 - protein, 9 aa, synthetic construct
GGGGQDQLR

SEQ ID NO: 43353 - protein, 9 aa, synthetic construct
GGGGQDQLT

SEQ ID NO: 43354 - protein, 9 aa, synthetic construct
GGGGQDRLE

SEQ ID NO: 43355 - protein, 9 aa, synthetic construct
GGGGQDRLF

SEQ ID NO: 43356 - protein, 9 aa, synthetic construct
GGGGQDRLK

SEQ ID NO: 43357 - protein, 9 aa, synthetic construct
GGGGQDRLM

SEQ ID NO: 43358 - protein, 9 aa, synthetic construct
GGGGQDRLY

SEQ ID NO: 43359 - protein, 9 aa, synthetic construct
GGGGQDRMI

SEQ ID NO: 43360 - protein, 9 aa, synthetic construct
GGGGQDSLF

SEQ ID NO: 43361 - protein, 9 aa, synthetic construct
GGGGQDSLH

SEQ ID NO: 43362 - protein, 9 aa, synthetic construct
GGGGQDSMF

SEQ ID NO: 43363 - protein, 9 aa, synthetic construct
GGGGQDTLV

SEQ ID NO: 43364 - protein, 9 aa, synthetic construct
GGGGQDTAD

SEQ ID NO: 43365 - protein, 9 aa, synthetic construct
GGGGQDTAH

SEQ ID NO: 43366 - protein, 9 aa, synthetic construct
GGGGQDTAI

SEQ ID NO: 43367 - protein, 9 aa, synthetic construct
GGGGQDTAS

SEQ ID NO: 43368 - protein, 9 aa, synthetic construct
GGGGQDTFL

SEQ ID NO: 43369 - protein, 9 aa, synthetic construct
GGGGQDTFN

SEQ ID NO: 43370 - protein, 9 aa, synthetic construct
GGGGQDTFY

SEQ ID NO: 43371 - protein, 9 aa, synthetic construct
GGGGQDTIG

SEQ ID NO: 43372 - protein, 9 aa, synthetic construct
GGGGQDTIL

SEQ ID NO: 43373 - protein, 9 aa, synthetic construct
GGGGQDTIW

SEQ ID NO: 43374 - protein, 9 aa, synthetic construct
GGGGQDTLE

SEQ ID NO: 43375 - protein, 9 aa, synthetic construct
GGGGQDTLK

SEQ ID NO: 43376 - protein, 9 aa, synthetic construct
GGGGQDTLQ

SEQ ID NO: 43377 - protein, 9 aa, synthetic construct
GGGGRDHLL

SEQ ID NO: 43378 - protein, 9 aa, synthetic construct
GGGGRDHLN

SEQ ID NO: 43379 - protein, 9 aa, synthetic construct
GGGGRDHLS

SEQ ID NO: 43380 - protein, 9 aa, synthetic construct
GGGGRDRFI

SEQ ID NO: 43381 - protein, 9 aa, synthetic construct
GGGGRDNLA

SEQ ID NO: 43382 - protein, 9 aa, synthetic construct
GGGGRDNLI

SEQ ID NO: 43383 - protein, 9 aa, synthetic construct
GGGGRDNLQ

SEQ ID NO: 43384 - protein, 9 aa, synthetic construct
GGGGRDQAD

SEQ ID NO: 43385 - protein, 9 aa, synthetic construct
GGGGRDQFL

SEQ ID NO: 43386 - protein, 9 aa, synthetic construct
GGGGRDQFV

SEQ ID NO: 43387 - protein, 9 aa, synthetic construct
GGGGRDQIR

SEQ ID NO: 43388 - protein, 9 aa, synthetic construct
GGGGRDQIS

SEQ ID NO: 43389 - protein, 9 aa, synthetic construct
GGGGRDQLA

SEQ ID NO: 43390 - protein, 9 aa, synthetic construct
GGGGRDQLI

SEQ ID NO: 43391 - protein, 9 aa, synthetic construct
GGGGRDQLN

SEQ ID NO: 43392 - protein, 9 aa, synthetic construct
GGGGRDQMA

SEQ ID NO: 43393 - protein, 9 aa, synthetic construct
GGGGRDRFE

SEQ ID NO: 43394 - protein, 9 aa, synthetic construct
GGGGRDRIL

SEQ ID NO: 43395 - protein, 9 aa, synthetic construct
GGGGRDMLW

SEQ ID NO: 43396 - protein, 9 aa, synthetic construct
GGGGRDRIQ

SEQ ID NO: 43397 - protein, 9 aa, synthetic construct
GGGGRDRIY

SEQ ID NO: 43398 - protein, 9 aa, synthetic construct
GGGGRDRLH

SEQ ID NO: 43399 - protein, 9 aa, synthetic construct
GGGGRDRLQ

SEQ ID NO: 43400 - protein, 9 aa, synthetic construct
GGGGRDRVD

SEQ ID NO: 43401 - protein, 9 aa, synthetic construct
GGGGRDRVN

SEQ ID NO: 43402 - protein, 9 aa, synthetic construct
GGGGRDRYV

SEQ ID NO: 43403 - protein, 9 aa, synthetic construct
GGGGRDSFL

SEQ ID NO: 43404 - protein, 9 aa, synthetic construct
GGGGRDSLD

SEQ ID NO: 43405 - protein, 9 aa, synthetic construct
GGGGRDSLH

SEQ ID NO: 43406 - protein, 9 aa, synthetic construct
GGGGRDSLL

SEQ ID NO: 43407 - protein, 9 aa, synthetic construct
GGGGRDSLV

SEQ ID NO: 43408 - protein, 9 aa, synthetic construct
GGGGRDTIG

SEQ ID NO: 43409 - protein, 9 aa, synthetic construct
GGGGRDNIR

SEQ ID NO: 43410 - protein, 9 aa, synthetic construct
GGGGRDMLG

SEQ ID NO: 43411 - protein, 9 aa, synthetic construct
GGGGRDHLY

SEQ ID NO: 43412 - protein, 9 aa, synthetic construct
GGGGRDKLV

SEQ ID NO: 43413 - protein, 9 aa, synthetic construct
GGGGRDHMF

SEQ ID NO: 43414 - protein, 9 aa, synthetic construct
GGGGRDIFD

SEQ ID NO: 43415 - protein, 9 aa, synthetic construct
GGGGRDIIS

SEQ ID NO: 43416 - protein, 9 aa, synthetic construct
GGGGRDILE

SEQ ID NO: 43417 - protein, 9 aa, synthetic construct
GGGGRDILL

SEQ ID NO: 43418 - protein, 9 aa, synthetic construct
GGGGRDILM

SEQ ID NO: 43419 - protein, 9 aa, synthetic construct
GGGGRDILT

SEQ ID NO: 43420 - protein, 9 aa, synthetic construct
GGGGRDIMT

SEQ ID NO: 43421 - protein, 9 aa, synthetic construct
GGGGRDIYV

SEQ ID NO: 43422 - protein, 9 aa, synthetic construct
GGGGRDKIA

SEQ ID NO: 43423 - protein, 9 aa, synthetic construct
GGGGRDKIL

SEQ ID NO: 43424 - protein, 9 aa, synthetic construct
GGGGRDKLD

SEQ ID NO: 43425 - protein, 9 aa, synthetic construct
GGGGRDKLS

SEQ ID NO: 43426 - protein, 9 aa, synthetic construct
GGGGRDLFI

SEQ ID NO: 43427 - protein, 9 aa, synthetic construct
GGGGRDMLD

SEQ ID NO: 43428 - protein, 9 aa, synthetic construct
GGGGRDLID

SEQ ID NO: 43429 - protein, 9 aa, synthetic construct
GGGGRDLIE

SEQ ID NO: 43430 - protein, 9 aa, synthetic construct
GGGGRDLIF

SEQ ID NO: 43431 - protein, 9 aa, synthetic construct
GGGGRDLIK

SEQ ID NO: 43432 - protein, 9 aa, synthetic construct
GGGGRDLIS

SEQ ID NO: 43433 - protein, 9 aa, synthetic construct
GGGGRDLLE

SEQ ID NO: 43434 - protein, 9 aa, synthetic construct
GGGGRDLLK

SEQ ID NO: 43435 - protein, 9 aa, synthetic construct
GGGGRDLLY

SEQ ID NO: 43436 - protein, 9 aa, synthetic construct
GGGGRDLMD

SEQ ID NO: 43437 - protein, 9 aa, synthetic construct
GGGGRDLMG

SEQ ID NO: 43438 - protein, 9 aa, synthetic construct
GGGGRDLVD

SEQ ID NO: 43439 - protein, 9 aa, synthetic construct
GGGGRDLVQ

SEQ ID NO: 43440 - protein, 9 aa, synthetic construct
GGGGRDMAD

SEQ ID NO: 43441 - protein, 9 aa, synthetic construct
GGHGNDVLE

SEQ ID NO: 43442 - protein, 9 aa, synthetic construct
GGHGNDVLL

SEQ ID NO: 43443 - protein, 9 aa, synthetic construct
GGHGNDVLR

SEQ ID NO: 43444 - protein, 9 aa, synthetic construct
GGIGQDIIY

SEQ ID NO: 43445 - protein, 9 aa, synthetic construct
GGIGNDVLF

SEQ ID NO: 43446 - protein, 9 aa, synthetic construct
GGIGNDVLK

SEQ ID NO: 43447 - protein, 9 aa, synthetic construct
GGIGNDVMH

SEQ ID NO: 43448 - protein, 9 aa, synthetic construct
GGIGNDVMN

SEQ ID NO: 43449 - protein, 9 aa, synthetic construct
GGIGNDVMS

SEQ ID NO: 43450 - protein, 9 aa, synthetic construct
GGIGNDVVA

SEQ ID NO: 43451 - protein, 9 aa, synthetic construct
GGIGNDVVL

SEQ ID NO: 43452 - protein, 9 aa, synthetic construct
GGIGNDVYA

SEQ ID NO: 43453 - protein, 9 aa, synthetic construct
GGIGNDVYF

SEQ ID NO: 43454 - protein, 9 aa, synthetic construct
GGIGNDVYL

SEQ ID NO: 43455 - protein, 9 aa, synthetic construct
GGIGNDWFR

SEQ ID NO: 43456 - protein, 9 aa, synthetic construct
GGIGNDWLA

SEQ ID NO: 43457 - protein, 9 aa, synthetic construct
GGIGNDWLE

SEQ ID NO: 43458 - protein, 9 aa, synthetic construct
GGIGNDWLF

SEQ ID NO: 43459 - protein, 9 aa, synthetic construct
GGIGNDWVG

SEQ ID NO: 43460 - protein, 9 aa, synthetic construct
GGIGNDYLH

SEQ ID NO: 43461 - protein, 9 aa, synthetic construct
GGIGNDYLI

SEQ ID NO: 43462 - protein, 9 aa, synthetic construct
GGIGNDYLQ

SEQ ID NO: 43463 - protein, 9 aa, synthetic construct
GGIGNDYMA

SEQ ID NO: 43464 - protein, 9 aa, synthetic construct
GGIGPDLLD

SEQ ID NO: 43465 - protein, 9 aa, synthetic construct
GGIGPDQMI

SEQ ID NO: 43466 - protein, 9 aa, synthetic construct
GGIGPDSLA

SEQ ID NO: 43467 - protein, 9 aa, synthetic construct
GGIGPDTLA

SEQ ID NO: 43468 - protein, 9 aa, synthetic construct
GGIGPDYLE

SEQ ID NO: 43469 - protein, 9 aa, synthetic construct
GGIGQDDLN

SEQ ID NO: 43470 - protein, 9 aa, synthetic construct
GGIGQDFLY

SEQ ID NO: 43471 - protein, 9 aa, synthetic construct
GGIGQDIFA

SEQ ID NO: 43472 - protein, 9 aa, synthetic construct
GGIGQDIFV

SEQ ID NO: 43473 - protein, 9 aa, synthetic construct
GGIGQDIIT

SEQ ID NO: 43474 - protein, 9 aa, synthetic construct
GGIGNDVIQ

SEQ ID NO: 43475 - protein, 9 aa, synthetic construct
GGIGNDVIK

SEQ ID NO: 43476 - protein, 9 aa, synthetic construct
GGIGNDVFT

SEQ ID NO: 43477 - protein, 9 aa, synthetic construct
GGIGNDTFR

SEQ ID NO: 43478 - protein, 9 aa, synthetic construct
GGIGNDSMA

SEQ ID NO: 43479 - protein, 9 aa, synthetic construct
GGIGNDSMR

SEQ ID NO: 43480 - protein, 9 aa, synthetic construct
GGIGNDSMT

SEQ ID NO: 43481 - protein, 9 aa, synthetic construct
GGIGNDSVD

SEQ ID NO: 43482 - protein, 9 aa, synthetic construct
GGIGNDSVG

SEQ ID NO: 43483 - protein, 9 aa, synthetic construct
GGIGNDSVL

SEQ ID NO: 43484 - protein, 9 aa, synthetic construct
GGIGNDSVY

SEQ ID NO: 43485 - protein, 9 aa, synthetic construct
GGIGNDSYL

SEQ ID NO: 43486 - protein, 9 aa, synthetic construct
GGIGNDTAD

SEQ ID NO: 43487 - protein, 9 aa, synthetic construct
GGIGNDTAN

SEQ ID NO: 43488 - protein, 9 aa, synthetic construct
GGIGNDTFF

SEQ ID NO: 43489 - protein, 9 aa, synthetic construct
GGIGNDTFN

SEQ ID NO: 43490 - protein, 9 aa, synthetic construct
GGIGNDTFQ

SEQ ID NO: 43491 - protein, 9 aa, synthetic construct
GGIGNDTFY

SEQ ID NO: 43492 - protein, 9 aa, synthetic construct
GGIGNDVFK

SEQ ID NO: 43493 - protein, 9 aa, synthetic construct
GGIGNDTIK

SEQ ID NO: 43494 - protein, 9 aa, synthetic construct
GGIGNDTLC

SEQ ID NO: 43495 - protein, 9 aa, synthetic construct
GGIGNDTLH

SEQ ID NO: 43496 - protein, 9 aa, synthetic construct
GGIGNDTLW

SEQ ID NO: 43497 - protein, 9 aa, synthetic construct
GGIGNDTVF

SEQ ID NO: 43498 - protein, 9 aa, synthetic construct
GGIGNDTVG

SEQ ID NO: 43499 - protein, 9 aa, synthetic construct
GGIGNDTVI

SEQ ID NO: 43500 - protein, 9 aa, synthetic construct
GGIGNDTVN

SEQ ID NO: 43501 - protein, 9 aa, synthetic construct
GGIGNDTVW

SEQ ID NO: 43502 - protein, 9 aa, synthetic construct
GGIGNDTYL

SEQ ID NO: 43503 - protein, 9 aa, synthetic construct
GGIGNDTYY

SEQ ID NO: 43504 - protein, 9 aa, synthetic construct
GGIGNDVAA

SEQ ID NO: 43505 - protein, 9 aa, synthetic construct
GGIGNDVAV

SEQ ID NO: 43506 - protein, 9 aa, synthetic construct
GGIGQDIIV

SEQ ID NO: 43507 - protein, 9 aa, synthetic construct
GGIGQDILA

SEQ ID NO: 43508 - protein, 9 aa, synthetic construct
GGIGRDVVD

SEQ ID NO: 43509 - protein, 9 aa, synthetic construct
GGIGQDILR

SEQ ID NO: 43510 - protein, 9 aa, synthetic construct
GGIGRDQID

SEQ ID NO: 43511 - protein, 9 aa, synthetic construct
GGIGRDQIN

SEQ ID NO: 43512 - protein, 9 aa, synthetic construct
GGIGRDQLA

SEQ ID NO: 43513 - protein, 9 aa, synthetic construct
GGIGRDQLY

SEQ ID NO: 43514 - protein, 9 aa, synthetic construct
GGIGRDRAS

SEQ ID NO: 43515 - protein, 9 aa, synthetic construct
GGIGRDRFW

SEQ ID NO: 43516 - protein, 9 aa, synthetic construct
GGIGRDRID

SEQ ID NO: 43517 - protein, 9 aa, synthetic construct
GGIGRDRLE

SEQ ID NO: 43518 - protein, 9 aa, synthetic construct
GGIGRDRLF

SEQ ID NO: 43519 - protein, 9 aa, synthetic construct
GGIGRDRLY

SEQ ID NO: 43520 - protein, 9 aa, synthetic construct
GGIGRDRMS

SEQ ID NO: 43521 - protein, 9 aa, synthetic construct
GGIGRDRVS

SEQ ID NO: 43522 - protein, 9 aa, synthetic construct
GGIGRDSLF

SEQ ID NO: 43523 - protein, 9 aa, synthetic construct
GGIGRDSVS

SEQ ID NO: 43524 - protein, 9 aa, synthetic construct
GGIGRDTIS

SEQ ID NO: 43525 - protein, 9 aa, synthetic construct
GGIGRDTLA

SEQ ID NO: 43526 - protein, 9 aa, synthetic construct
GGIGRDTLL

SEQ ID NO: 43527 - protein, 9 aa, synthetic construct
GGIGRDTLR

SEQ ID NO: 43528 - protein, 9 aa, synthetic construct
GGIGRDTMF

SEQ ID NO: 43529 - protein, 9 aa, synthetic construct
GGIGRDTMT

SEQ ID NO: 43530 - protein, 9 aa, synthetic construct
GGIGRDTYV

SEQ ID NO: 43531 - protein, 9 aa, synthetic construct
GGIGRDTYW

SEQ ID NO: 43532 - protein, 9 aa, synthetic construct
GGIGRDVAS

SEQ ID NO: 43533 - protein, 9 aa, synthetic construct
GGIGRDVID

SEQ ID NO: 43534 - protein, 9 aa, synthetic construct
GGIGRDVLI

SEQ ID NO: 43535 - protein, 9 aa, synthetic construct
GGIGRDVLK

SEQ ID NO: 43536 - protein, 9 aa, synthetic construct
GGIGRDVLN

SEQ ID NO: 43537 - protein, 9 aa, synthetic construct
GGIGRDVLT

SEQ ID NO: 43538 - protein, 9 aa, synthetic construct
GGIGRDVLY

SEQ ID NO: 43539 - protein, 9 aa, synthetic construct
GGIGRDNLF

SEQ ID NO: 43540 - protein, 9 aa, synthetic construct
GGIGRDLIF

SEQ ID NO: 43541 - protein, 9 aa, synthetic construct
GGIGRDLFG

SEQ ID NO: 43542 - protein, 9 aa, synthetic construct
GGIGQDTLV

SEQ ID NO: 43543 - protein, 9 aa, synthetic construct
GGIGQDILS

SEQ ID NO: 43544 - protein, 9 aa, synthetic construct
GGIGQDLLV

SEQ ID NO: 43545 - protein, 9 aa, synthetic construct
GGIGQDLVE

SEQ ID NO: 43546 - protein, 9 aa, synthetic construct
GGIGQDRFL

SEQ ID NO: 43547 - protein, 9 aa, synthetic construct
GGIGQDRFS

SEQ ID NO: 43548 - protein, 9 aa, synthetic construct
GGIGQDRLL

SEQ ID NO: 43549 - protein, 9 aa, synthetic construct
GGIGQDRMI

SEQ ID NO: 43550 - protein, 9 aa, synthetic construct
GGIGQDRMV

SEQ ID NO: 43551 - protein, 9 aa, synthetic construct
GGIGQDSLT

SEQ ID NO: 43552 - protein, 9 aa, synthetic construct
GGIGQDTID

SEQ ID NO: 43553 - protein, 9 aa, synthetic construct
GGIGQDTLF

SEQ ID NO: 43554 - protein, 9 aa, synthetic construct
GGIGQDTLI

SEQ ID NO: 43555 - protein, 9 aa, synthetic construct
GGIGQDTLL

SEQ ID NO: 43556 - protein, 9 aa, synthetic construct
GGIGQDTLW

SEQ ID NO: 43557 - protein, 9 aa, synthetic construct
GGIGRDKLY

SEQ ID NO: 43558 - protein, 9 aa, synthetic construct
GGIGQDTLY

SEQ ID NO: 43559 - protein, 9 aa, synthetic construct
GGIGQDVLT

SEQ ID NO: 43560 - protein, 9 aa, synthetic construct
GGIGQDVLV

SEQ ID NO: 43561 - protein, 9 aa, synthetic construct
GGIGQDVVD

SEQ ID NO: 43562 - protein, 9 aa, synthetic construct
GGIGRDAIS

SEQ ID NO: 43563 - protein, 9 aa, synthetic construct
GGIGRDDLI

SEQ ID NO: 43564 - protein, 9 aa, synthetic construct
GGIGRDFLV

SEQ ID NO: 43565 - protein, 9 aa, synthetic construct
GGIGRDGLN

SEQ ID NO: 43566 - protein, 9 aa, synthetic construct
GGIGRDIFA

SEQ ID NO: 43567 - protein, 9 aa, synthetic construct
GGIGRDILT

SEQ ID NO: 43568 - protein, 9 aa, synthetic construct
GGIGRDKID

SEQ ID NO: 43569 - protein, 9 aa, synthetic construct
GGIGRDKIR

SEQ ID NO: 43570 - protein, 9 aa, synthetic construct
GGIGRDKLA

SEQ ID NO: 43571 - protein, 9 aa, synthetic construct
GGIGNDSLC

SEQ ID NO: 43572 - protein, 9 aa, synthetic construct
GGIGNDSLA

SEQ ID NO: 43573 - protein, 9 aa, synthetic construct
GGIGNDSIS

SEQ ID NO: 43574 - protein, 9 aa, synthetic construct
GGIGNDSIH

SEQ ID NO: 43575 - protein, 9 aa, synthetic construct
GGIGNDFLL

SEQ ID NO: 43576 - protein, 9 aa, synthetic construct
GGIGNDFLQ

SEQ ID NO: 43577 - protein, 9 aa, synthetic construct
GGIGNDGIY

SEQ ID NO: 43578 - protein, 9 aa, synthetic construct
GGIGNDGVF

SEQ ID NO: 43579 - protein, 9 aa, synthetic construct
GGIGNDGYV

SEQ ID NO: 43580 - protein, 9 aa, synthetic construct
GGIGNDGYY

SEQ ID NO: 43581 - protein, 9 aa, synthetic construct
GGIGNDHLD

SEQ ID NO: 43582 - protein, 9 aa, synthetic construct
GGIGNDHLS

SEQ ID NO: 43583 - protein, 9 aa, synthetic construct
GGIGNDIFI

SEQ ID NO: 43584 - protein, 9 aa, synthetic construct
GGIGNDIFV

SEQ ID NO: 43585 - protein, 9 aa, synthetic construct
GGIGNDIIC

SEQ ID NO: 43586 - protein, 9 aa, synthetic construct
GGIGNDIII

SEQ ID NO: 43587 - protein, 9 aa, synthetic construct
GGIGNDIIL

SEQ ID NO: 43588 - protein, 9 aa, synthetic construct
GGIGNDIIM

SEQ ID NO: 43589 - protein, 9 aa, synthetic construct
GGIGNDIIQ

SEQ ID NO: 43590 - protein, 9 aa, synthetic construct
GGIGNDIIV

SEQ ID NO: 43591 - protein, 9 aa, synthetic construct
GGIGNDIIY

SEQ ID NO: 43592 - protein, 9 aa, synthetic construct
GGIGNDILG

SEQ ID NO: 43593 - protein, 9 aa, synthetic construct
GGIGNDILH

SEQ ID NO: 43594 - protein, 9 aa, synthetic construct
GGIGNDILK

SEQ ID NO: 43595 - protein, 9 aa, synthetic construct
GGIGNDILW

SEQ ID NO: 43596 - protein, 9 aa, synthetic construct
GGIGNDIMT

SEQ ID NO: 43597 - protein, 9 aa, synthetic construct
GGIGNDIVD

SEQ ID NO: 43598 - protein, 9 aa, synthetic construct
GGIGNDIVN

SEQ ID NO: 43599 - protein, 9 aa, synthetic construct
GGIGNDIYN

SEQ ID NO: 43600 - protein, 9 aa, synthetic construct
GGIGNDIYT

SEQ ID NO: 43601 - protein, 9 aa, synthetic construct
GGIGNDKIA

SEQ ID NO: 43602 - protein, 9 aa, synthetic construct
GGIGNDKIS

SEQ ID NO: 43603 - protein, 9 aa, synthetic construct
GGIGNDKIT

SEQ ID NO: 43604 - protein, 9 aa, synthetic construct
GGIGNDFLI

SEQ ID NO: 43605 - protein, 9 aa, synthetic construct
GGIGNDFIT

SEQ ID NO: 43606 - protein, 9 aa, synthetic construct
GGIGNDFIF

SEQ ID NO: 43607 - protein, 9 aa, synthetic construct
GGIGNDDIF

SEQ ID NO: 43608 - protein, 9 aa, synthetic construct
GGIGMDWMR

SEQ ID NO: 43609 - protein, 9 aa, synthetic construct
GGIGNDAID

SEQ ID NO: 43610 - protein, 9 aa, synthetic construct
GGIGNDAIF

SEQ ID NO: 43611 - protein, 9 aa, synthetic construct
GGIGNDAIQ

SEQ ID NO: 43612 - protein, 9 aa, synthetic construct
GGIGNDALH

SEQ ID NO: 43613 - protein, 9 aa, synthetic construct
GGIGNDALI

SEQ ID NO: 43614 - protein, 9 aa, synthetic construct
GGIGNDALV

SEQ ID NO: 43615 - protein, 9 aa, synthetic construct
GGIGNDALW

SEQ ID NO: 43616 - protein, 9 aa, synthetic construct
GGIGNDAMT

SEQ ID NO: 43617 - protein, 9 aa, synthetic construct
GGIGNDAVR

SEQ ID NO: 43618 - protein, 9 aa, synthetic construct
GGIGNDAVS

SEQ ID NO: 43619 - protein, 9 aa, synthetic construct
GGIGNDAYV

SEQ ID NO: 43620 - protein, 9 aa, synthetic construct
GGIGNDDID

SEQ ID NO: 43621 - protein, 9 aa, synthetic construct
GGIGNDDIK

SEQ ID NO: 43622 - protein, 9 aa, synthetic construct
GGIGNDFID

SEQ ID NO: 43623 - protein, 9 aa, synthetic construct
GGIGNDDLA

SEQ ID NO: 43624 - protein, 9 aa, synthetic construct
GGIGNDDLH

SEQ ID NO: 43625 - protein, 9 aa, synthetic construct
GGIGNDDLL

SEQ ID NO: 43626 - protein, 9 aa, synthetic construct
GGIGNDDLT

SEQ ID NO: 43627 - protein, 9 aa, synthetic construct
GGIGNDDLY

SEQ ID NO: 43628 - protein, 9 aa, synthetic construct
GGIGNDEAE

SEQ ID NO: 43629 - protein, 9 aa, synthetic construct
GGIGNDEID

SEQ ID NO: 43630 - protein, 9 aa, synthetic construct
GGIGNDEIH

SEQ ID NO: 43631 - protein, 9 aa, synthetic construct
GGIGNDELM

SEQ ID NO: 43632 - protein, 9 aa, synthetic construct
GGIGNDEYR

SEQ ID NO: 43633 - protein, 9 aa, synthetic construct
GGIGNDFAF

SEQ ID NO: 43634 - protein, 9 aa, synthetic construct
GGIGNDFAN

SEQ ID NO: 43635 - protein, 9 aa, synthetic construct
GGIGNDFFS

SEQ ID NO: 43636 - protein, 9 aa, synthetic construct
GGIGNDKLL

SEQ ID NO: 43637 - protein, 9 aa, synthetic construct
GGIGNDKLN

SEQ ID NO: 43638 - protein, 9 aa, synthetic construct
GGIGNDKLR

SEQ ID NO: 43639 - protein, 9 aa, synthetic construct
GGIGNDRMF

SEQ ID NO: 43640 - protein, 9 aa, synthetic construct
GGIGNDQIG

SEQ ID NO: 43641 - protein, 9 aa, synthetic construct
GGIGNDQLH

SEQ ID NO: 43642 - protein, 9 aa, synthetic construct
GGIGNDQLI

SEQ ID NO: 43643 - protein, 9 aa, synthetic construct
GGIGNDQLL

SEQ ID NO: 43644 - protein, 9 aa, synthetic construct
GGIGNDQLQ

SEQ ID NO: 43645 - protein, 9 aa, synthetic construct
GGIGNDQVS

SEQ ID NO: 43646 - protein, 9 aa, synthetic construct
GGIGNDRFV

SEQ ID NO: 43647 - protein, 9 aa, synthetic construct
GGIGNDRID

SEQ ID NO: 43648 - protein, 9 aa, synthetic construct
GGIGNDRII

SEQ ID NO: 43649 - protein, 9 aa, synthetic construct
GGIGNDRIL

SEQ ID NO: 43650 - protein, 9 aa, synthetic construct
GGIGNDRIQ

SEQ ID NO: 43651 - protein, 9 aa, synthetic construct
GGIGNDRIS

SEQ ID NO: 43652 - protein, 9 aa, synthetic construct
GGIGNDRMD

SEQ ID NO: 43653 - protein, 9 aa, synthetic construct
GGIGNDRMN

SEQ ID NO: 43654 - protein, 9 aa, synthetic construct
GGIGNDNVD

SEQ ID NO: 43655 - protein, 9 aa, synthetic construct
GGIGNDRMQ

SEQ ID NO: 43656 - protein, 9 aa, synthetic construct
GGIGNDRMS

SEQ ID NO: 43657 - protein, 9 aa, synthetic construct
GGIGNDRMT

SEQ ID NO: 43658 - protein, 9 aa, synthetic construct
GGIGNDRVK

SEQ ID NO: 43659 - protein, 9 aa, synthetic construct
GGIGNDRVS

SEQ ID NO: 43660 - protein, 9 aa, synthetic construct
GGIGNDRVY

SEQ ID NO: 43661 - protein, 9 aa, synthetic construct
GGIGNDRYI

SEQ ID NO: 43662 - protein, 9 aa, synthetic construct
GGIGNDSAL

SEQ ID NO: 43663 - protein, 9 aa, synthetic construct
GGIGNDSAM

SEQ ID NO: 43664 - protein, 9 aa, synthetic construct
GGIGNDSAW

SEQ ID NO: 43665 - protein, 9 aa, synthetic construct
GGIGNDSFI

SEQ ID NO: 43666 - protein, 9 aa, synthetic construct
GGIGNDSIE

SEQ ID NO: 43667 - protein, 9 aa, synthetic construct
GGIGNDSIF

SEQ ID NO: 43668 - protein, 9 aa, synthetic construct
GGIGNDQID

SEQ ID NO: 43669 - protein, 9 aa, synthetic construct
GGIGNDNLT

SEQ ID NO: 43670 - protein, 9 aa, synthetic construct
GGIGNDKLV

SEQ ID NO: 43671 - protein, 9 aa, synthetic construct
GGIGNDLVS

SEQ ID NO: 43672 - protein, 9 aa, synthetic construct
GGIGNDLIG

SEQ ID NO: 43673 - protein, 9 aa, synthetic construct
GGIGNDLII

SEQ ID NO: 43674 - protein, 9 aa, synthetic construct
GGIGNDLIL

SEQ ID NO: 43675 - protein, 9 aa, synthetic construct
GGIGNDLIN

SEQ ID NO: 43676 - protein, 9 aa, synthetic construct
GGIGNDLIQ

SEQ ID NO: 43677 - protein, 9 aa, synthetic construct
GGIGNDLLA

SEQ ID NO: 43678 - protein, 9 aa, synthetic construct
GGIGNDLLG

SEQ ID NO: 43679 - protein, 9 aa, synthetic construct
GGIGNDLLK

SEQ ID NO: 43680 - protein, 9 aa, synthetic construct
GGIGNDLLM

SEQ ID NO: 43681 - protein, 9 aa, synthetic construct
GGIGNDLLR

SEQ ID NO: 43682 - protein, 9 aa, synthetic construct
GGIGNDLLW

SEQ ID NO: 43683 - protein, 9 aa, synthetic construct
GGIGNDLMH

SEQ ID NO: 43684 - protein, 9 aa, synthetic construct
GGIGNDLVR

SEQ ID NO: 43685 - protein, 9 aa, synthetic construct
GGIGNDLYI

SEQ ID NO: 43686 - protein, 9 aa, synthetic construct
GGIGNDNLS

SEQ ID NO: 43687 - protein, 9 aa, synthetic construct
GGIGNDLYL

SEQ ID NO: 43688 - protein, 9 aa, synthetic construct
GGIGNDLYR

SEQ ID NO: 43689 - protein, 9 aa, synthetic construct
GGIGNDMAE

SEQ ID NO: 43690 - protein, 9 aa, synthetic construct
GGIGNDMID

SEQ ID NO: 43691 - protein, 9 aa, synthetic construct
GGIGNDMIF

SEQ ID NO: 43692 - protein, 9 aa, synthetic construct
GGIGNDMIN

SEQ ID NO: 43693 - protein, 9 aa, synthetic construct
GGIGNDMLK

SEQ ID NO: 43694 - protein, 9 aa, synthetic construct
GGIGNDMLS

SEQ ID NO: 43695 - protein, 9 aa, synthetic construct
GGIGNDMLV

SEQ ID NO: 43696 - protein, 9 aa, synthetic construct
GGIGNDMLY

SEQ ID NO: 43697 - protein, 9 aa, synthetic construct
GGIGNDNFQ

SEQ ID NO: 43698 - protein, 9 aa, synthetic construct
GGIGNDNIY

SEQ ID NO: 43699 - protein, 9 aa, synthetic construct
GGIGNDNLM

SEQ ID NO: 43700 - protein, 9 aa, synthetic construct
GGIGRDVMT

SEQ ID NO: 43701 - protein, 9 aa, synthetic construct
GGIGRDWLD

SEQ ID NO: 43702 - protein, 9 aa, synthetic construct
GGHGNDVMF

SEQ ID NO: 43703 - protein, 9 aa, synthetic construct
GGKGADQLR

SEQ ID NO: 43704 - protein, 9 aa, synthetic construct
GGKGADILV

SEQ ID NO: 43705 - protein, 9 aa, synthetic construct
GGKGADIMD

SEQ ID NO: 43706 - protein, 9 aa, synthetic construct
GGKGADIMQ

SEQ ID NO: 43707 - protein, 9 aa, synthetic construct
GGKGADIMT

SEQ ID NO: 43708 - protein, 9 aa, synthetic construct
GGKGADIYL

SEQ ID NO: 43709 - protein, 9 aa, synthetic construct
GGKGADKAD

SEQ ID NO: 43710 - protein, 9 aa, synthetic construct
GGKGADKIF

SEQ ID NO: 43711 - protein, 9 aa, synthetic construct
GGKGADKIQ

SEQ ID NO: 43712 - protein, 9 aa, synthetic construct
GGKGADKLD

SEQ ID NO: 43713 - protein, 9 aa, synthetic construct
GGKGADKLE

SEQ ID NO: 43714 - protein, 9 aa, synthetic construct
GGKGADLIE

SEQ ID NO: 43715 - protein, 9 aa, synthetic construct
GGKGADLIQ

SEQ ID NO: 43716 - protein, 9 aa, synthetic construct
GGKGADLIV

SEQ ID NO: 43717 - protein, 9 aa, synthetic construct
GGKGADLLQ

SEQ ID NO: 43718 - protein, 9 aa, synthetic construct
GGKGADLLR

SEQ ID NO: 43719 - protein, 9 aa, synthetic construct
GGKGADLYE

SEQ ID NO: 43720 - protein, 9 aa, synthetic construct
GGKGADMFI

SEQ ID NO: 43721 - protein, 9 aa, synthetic construct
GGKGADMLF

SEQ ID NO: 43722 - protein, 9 aa, synthetic construct
GGKGADMLI

SEQ ID NO: 43723 - protein, 9 aa, synthetic construct
GGKGADNFH

SEQ ID NO: 43724 - protein, 9 aa, synthetic construct
GGKGADNIY

SEQ ID NO: 43725 - protein, 9 aa, synthetic construct
GGKGADNLT

SEQ ID NO: 43726 - protein, 9 aa, synthetic construct
GGKGADQFI

SEQ ID NO: 43727 - protein, 9 aa, synthetic construct
GGKGADQFV

SEQ ID NO: 43728 - protein, 9 aa, synthetic construct
GGKGADQID

SEQ ID NO: 43729 - protein, 9 aa, synthetic construct
GGKGADQIL

SEQ ID NO: 43730 - protein, 9 aa, synthetic construct
GGKGADQIW

SEQ ID NO: 43731 - protein, 9 aa, synthetic construct
GGKGADQIY

SEQ ID NO: 43732 - protein, 9 aa, synthetic construct
GGKGADQLE

SEQ ID NO: 43733 - protein, 9 aa, synthetic construct
GGKGADILL

SEQ ID NO: 43734 - protein, 9 aa, synthetic construct
GGKGADILK

SEQ ID NO: 43735 - protein, 9 aa, synthetic construct
GGKGADIFA

SEQ ID NO: 43736 - protein, 9 aa, synthetic construct
GGKGADELW

SEQ ID NO: 43737 - protein, 9 aa, synthetic construct
GGKGADDIR

SEQ ID NO: 43738 - protein, 9 aa, synthetic construct
GGKGADDIY

SEQ ID NO: 43739 - protein, 9 aa, synthetic construct
GGKGADDLF

SEQ ID NO: 43740 - protein, 9 aa, synthetic construct
GGKGADDLL

SEQ ID NO: 43741 - protein, 9 aa, synthetic construct
GGKGADDMD

SEQ ID NO: 43742 - protein, 9 aa, synthetic construct
GGKGADDYI

SEQ ID NO: 43743 - protein, 9 aa, synthetic construct
GGKGADEFQ

SEQ ID NO: 43744 - protein, 9 aa, synthetic construct
GGKGADEIL

SEQ ID NO: 43745 - protein, 9 aa, synthetic construct
GGKGADELE

SEQ ID NO: 43746 - protein, 9 aa, synthetic construct
GGKGADELF

SEQ ID NO: 43747 - protein, 9 aa, synthetic construct
GGKGADELN

SEQ ID NO: 43748 - protein, 9 aa, synthetic construct
GGKGADELQ

SEQ ID NO: 43749 - protein, 9 aa, synthetic construct
GGKGADELV

SEQ ID NO: 43750 - protein, 9 aa, synthetic construct
GGKGADEMI

SEQ ID NO: 43751 - protein, 9 aa, synthetic construct
GGKGADHLF

SEQ ID NO: 43752 - protein, 9 aa, synthetic construct
GGKGADEMR

SEQ ID NO: 43753 - protein, 9 aa, synthetic construct
GGKGADFLA

SEQ ID NO: 43754 - protein, 9 aa, synthetic construct
GGKGADFLD

SEQ ID NO: 43755 - protein, 9 aa, synthetic construct
GGKGADFLQ

SEQ ID NO: 43756 - protein, 9 aa, synthetic construct
GGKGADFLW

SEQ ID NO: 43757 - protein, 9 aa, synthetic construct
GGKGADFMN

SEQ ID NO: 43758 - protein, 9 aa, synthetic construct
GGKGADFVD

SEQ ID NO: 43759 - protein, 9 aa, synthetic construct
GGKGADFVE

SEQ ID NO: 43760 - protein, 9 aa, synthetic construct
GGKGADFYD

SEQ ID NO: 43761 - protein, 9 aa, synthetic construct
GGKGADGFY

SEQ ID NO: 43762 - protein, 9 aa, synthetic construct
GGKGADGLY

SEQ ID NO: 43763 - protein, 9 aa, synthetic construct
GGKGADGVY

SEQ ID NO: 43764 - protein, 9 aa, synthetic construct
GGKGADHII

SEQ ID NO: 43765 - protein, 9 aa, synthetic construct
GGKGADQLI

SEQ ID NO: 43766 - protein, 9 aa, synthetic construct
GGKGADRFY

SEQ ID NO: 43767 - protein, 9 aa, synthetic construct
GGIGRDWLY

SEQ ID NO: 43768 - protein, 9 aa, synthetic construct
GGKGADRLL

SEQ ID NO: 43769 - protein, 9 aa, synthetic construct
GGKGADTVF

SEQ ID NO: 43770 - protein, 9 aa, synthetic construct
GGKGADTYR

SEQ ID NO: 43771 - protein, 9 aa, synthetic construct
GGKGADTYV

SEQ ID NO: 43772 - protein, 9 aa, synthetic construct
GGKGADVFC

SEQ ID NO: 43773 - protein, 9 aa, synthetic construct
GGKGADVFD

SEQ ID NO: 43774 - protein, 9 aa, synthetic construct
GGKGADVFI

SEQ ID NO: 43775 - protein, 9 aa, synthetic construct
GGKGADVFL

SEQ ID NO: 43776 - protein, 9 aa, synthetic construct
GGKGADVFN

SEQ ID NO: 43777 - protein, 9 aa, synthetic construct
GGKGADVID

SEQ ID NO: 43778 - protein, 9 aa, synthetic construct
GGKGADVIE

SEQ ID NO: 43779 - protein, 9 aa, synthetic construct
GGKGADVLF

SEQ ID NO: 43780 - protein, 9 aa, synthetic construct
GGKGADVLL

SEQ ID NO: 43781 - protein, 9 aa, synthetic construct
GGKGADVLQ

SEQ ID NO: 43782 - protein, 9 aa, synthetic construct
GGKGADVLS

SEQ ID NO: 43783 - protein, 9 aa, synthetic construct
GGKGADVLY

SEQ ID NO: 43784 - protein, 9 aa, synthetic construct
GGKGADVMV

SEQ ID NO: 43785 - protein, 9 aa, synthetic construct
GGKGADWLM

SEQ ID NO: 43786 - protein, 9 aa, synthetic construct
GGKGADWLN

SEQ ID NO: 43787 - protein, 9 aa, synthetic construct
GGKGADWLR

SEQ ID NO: 43788 - protein, 9 aa, synthetic construct
GGKGADYLE

SEQ ID NO: 43789 - protein, 9 aa, synthetic construct
GGKGADYLI

SEQ ID NO: 43790 - protein, 9 aa, synthetic construct
GGKGADYLY

SEQ ID NO: 43791 - protein, 9 aa, synthetic construct
GGKGDDAIE

SEQ ID NO: 43792 - protein, 9 aa, synthetic construct
GGKGDDALE

SEQ ID NO: 43793 - protein, 9 aa, synthetic construct
GGKGDDALF

SEQ ID NO: 43794 - protein, 9 aa, synthetic construct
GGKGDDALN

SEQ ID NO: 43795 - protein, 9 aa, synthetic construct
GGKGDDALS

SEQ ID NO: 43796 - protein, 9 aa, synthetic construct
GGKGDDAVH

SEQ ID NO: 43797 - protein, 9 aa, synthetic construct
GGKGDDAYI

SEQ ID NO: 43798 - protein, 9 aa, synthetic construct
GGKGADTVE

SEQ ID NO: 43799 - protein, 9 aa, synthetic construct
GGKGADTVD

SEQ ID NO: 43800 - protein, 9 aa, synthetic construct
GGKGADTMS

SEQ ID NO: 43801 - protein, 9 aa, synthetic construct
GGKGADSMY

SEQ ID NO: 43802 - protein, 9 aa, synthetic construct
GGKGADRLR

SEQ ID NO: 43803 - protein, 9 aa, synthetic construct
GGKGADRMA

SEQ ID NO: 43804 - protein, 9 aa, synthetic construct
GGKGADRME

SEQ ID NO: 43805 - protein, 9 aa, synthetic construct
GGKGADRMT

SEQ ID NO: 43806 - protein, 9 aa, synthetic construct
GGKGADRVD

SEQ ID NO: 43807 - protein, 9 aa, synthetic construct
GGKGADSFF

SEQ ID NO: 43808 - protein, 9 aa, synthetic construct
GGKGADSFL

SEQ ID NO: 43809 - protein, 9 aa, synthetic construct
GGKGADSID

SEQ ID NO: 43810 - protein, 9 aa, synthetic construct
GGKGADSLA

SEQ ID NO: 43811 - protein, 9 aa, synthetic construct
GGKGADSLN

SEQ ID NO: 43812 - protein, 9 aa, synthetic construct
GGKGADSLR

SEQ ID NO: 43813 - protein, 9 aa, synthetic construct
GGKGADSMA

SEQ ID NO: 43814 - protein, 9 aa, synthetic construct
GGKGADSMH

SEQ ID NO: 43815 - protein, 9 aa, synthetic construct
GGKGADSVV

SEQ ID NO: 43816 - protein, 9 aa, synthetic construct
GGKGADTMR

SEQ ID NO: 43817 - protein, 9 aa, synthetic construct
GGKGADTAN

SEQ ID NO: 43818 - protein, 9 aa, synthetic construct
GGKGADTFN

SEQ ID NO: 43819 - protein, 9 aa, synthetic construct
GGKGADTFT

SEQ ID NO: 43820 - protein, 9 aa, synthetic construct
GGKGADTIE

SEQ ID NO: 43821 - protein, 9 aa, synthetic construct
GGKGADTIL

SEQ ID NO: 43822 - protein, 9 aa, synthetic construct
GGKGADTIR

SEQ ID NO: 43823 - protein, 9 aa, synthetic construct
GGKGADTLE

SEQ ID NO: 43824 - protein, 9 aa, synthetic construct
GGKGADTLF

SEQ ID NO: 43825 - protein, 9 aa, synthetic construct
GGKGADTLK

SEQ ID NO: 43826 - protein, 9 aa, synthetic construct
GGKGADTLS

SEQ ID NO: 43827 - protein, 9 aa, synthetic construct
GGKGADTLY

SEQ ID NO: 43828 - protein, 9 aa, synthetic construct
GGKGADTMI

SEQ ID NO: 43829 - protein, 9 aa, synthetic construct
GGKGADTMN

SEQ ID NO: 43830 - protein, 9 aa, synthetic construct
GGKGADAME

SEQ ID NO: 43831 - protein, 9 aa, synthetic construct
GGKGADAMD

SEQ ID NO: 43832 - protein, 9 aa, synthetic construct
GGKGADALW

SEQ ID NO: 43833 - protein, 9 aa, synthetic construct
GGKGADALS

SEQ ID NO: 43834 - protein, 9 aa, synthetic construct
GGIGSDRFV

SEQ ID NO: 43835 - protein, 9 aa, synthetic construct
GGIGSDRIW

SEQ ID NO: 43836 - protein, 9 aa, synthetic construct
GGIGSDRLE

SEQ ID NO: 43837 - protein, 9 aa, synthetic construct
GGIGSDRLK

SEQ ID NO: 43838 - protein, 9 aa, synthetic construct
GGIGSDSIE

SEQ ID NO: 43839 - protein, 9 aa, synthetic construct
GGIGSDSIS

SEQ ID NO: 43840 - protein, 9 aa, synthetic construct
GGIGSDSLA

SEQ ID NO: 43841 - protein, 9 aa, synthetic construct
GGIGSDSLH

SEQ ID NO: 43842 - protein, 9 aa, synthetic construct
GGIGSDSLV

SEQ ID NO: 43843 - protein, 9 aa, synthetic construct
GGIGSDSMT

SEQ ID NO: 43844 - protein, 9 aa, synthetic construct
GGIGSDSMV

SEQ ID NO: 43845 - protein, 9 aa, synthetic construct
GGIGSDSVD

SEQ ID NO: 43846 - protein, 9 aa, synthetic construct
GGIGSDSYY

SEQ ID NO: 43847 - protein, 9 aa, synthetic construct
GGIGSDTAS

SEQ ID NO: 43848 - protein, 9 aa, synthetic construct
GGIGSDTAV

SEQ ID NO: 43849 - protein, 9 aa, synthetic construct
GGIGSDTIK

SEQ ID NO: 43850 - protein, 9 aa, synthetic construct
GGIGSDTLA

SEQ ID NO: 43851 - protein, 9 aa, synthetic construct
GGIGSDTLF

SEQ ID NO: 43852 - protein, 9 aa, synthetic construct
GGIGSDTLK

SEQ ID NO: 43853 - protein, 9 aa, synthetic construct
GGIGSDTLY

SEQ ID NO: 43854 - protein, 9 aa, synthetic construct
GGIGSDTMA

SEQ ID NO: 43855 - protein, 9 aa, synthetic construct
GGIGSDTMS

SEQ ID NO: 43856 - protein, 9 aa, synthetic construct
GGIGSDTVS

SEQ ID NO: 43857 - protein, 9 aa, synthetic construct
GGIGSDTYL

SEQ ID NO: 43858 - protein, 9 aa, synthetic construct
GGIGSDTYY

SEQ ID NO: 43859 - protein, 9 aa, synthetic construct
GGIGSDVAD

SEQ ID NO: 43860 - protein, 9 aa, synthetic construct
GGIGSDVID

SEQ ID NO: 43861 - protein, 9 aa, synthetic construct
GGIGSDVIN

SEQ ID NO: 43862 - protein, 9 aa, synthetic construct
GGIGSDVLE

SEQ ID NO: 43863 - protein, 9 aa, synthetic construct
GGIGSDRFL

SEQ ID NO: 43864 - protein, 9 aa, synthetic construct
GGIGSDQVY

SEQ ID NO: 43865 - protein, 9 aa, synthetic construct
GGIGSDQLY

SEQ ID NO: 43866 - protein, 9 aa, synthetic construct
GGIGSDIIH

SEQ ID NO: 43867 - protein, 9 aa, synthetic construct
GGIGRDYLD

SEQ ID NO: 43868 - protein, 9 aa, synthetic construct
GGIGRDYMA

SEQ ID NO: 43869 - protein, 9 aa, synthetic construct
GGIGSDALQ

SEQ ID NO: 43870 - protein, 9 aa, synthetic construct
GGIGSDAMS

SEQ ID NO: 43871 - protein, 9 aa, synthetic construct
GGIGSDDLG

SEQ ID NO: 43872 - protein, 9 aa, synthetic construct
GGIGSDDLY

SEQ ID NO: 43873 - protein, 9 aa, synthetic construct
GGIGSDEII

SEQ ID NO: 43874 - protein, 9 aa, synthetic construct
GGIGSDELS

SEQ ID NO: 43875 - protein, 9 aa, synthetic construct
GGIGSDELV

SEQ ID NO: 43876 - protein, 9 aa, synthetic construct
GGIGSDFLY

SEQ ID NO: 43877 - protein, 9 aa, synthetic construct
GGIGSDHLD

SEQ ID NO: 43878 - protein, 9 aa, synthetic construct
GGIGSDHLS

SEQ ID NO: 43879 - protein, 9 aa, synthetic construct
GGIGSDHVD

SEQ ID NO: 43880 - protein, 9 aa, synthetic construct
GGIGSDILF

SEQ ID NO: 43881 - protein, 9 aa, synthetic construct
GGIGSDQLT

SEQ ID NO: 43882 - protein, 9 aa, synthetic construct
GGIGSDILL

SEQ ID NO: 43883 - protein, 9 aa, synthetic construct
GGIGSDILT

SEQ ID NO: 43884 - protein, 9 aa, synthetic construct
GGIGSDILY

SEQ ID NO: 43885 - protein, 9 aa, synthetic construct
GGIGSDIVN

SEQ ID NO: 43886 - protein, 9 aa, synthetic construct
GGIGSDKLD

SEQ ID NO: 43887 - protein, 9 aa, synthetic construct
GGIGSDKLY

SEQ ID NO: 43888 - protein, 9 aa, synthetic construct
GGIGSDLLA

SEQ ID NO: 43889 - protein, 9 aa, synthetic construct
GGIGSDLLR

SEQ ID NO: 43890 - protein, 9 aa, synthetic construct
GGIGSDLLY

SEQ ID NO: 43891 - protein, 9 aa, synthetic construct
GGIGSDLMS

SEQ ID NO: 43892 - protein, 9 aa, synthetic construct
GGIGSDLMY

SEQ ID NO: 43893 - protein, 9 aa, synthetic construct
GGIGSDNLR

SEQ ID NO: 43894 - protein, 9 aa, synthetic construct
GGIGSDQLI

SEQ ID NO: 43895 - protein, 9 aa, synthetic construct
GGIGSDVLK

SEQ ID NO: 43896 - protein, 9 aa, synthetic construct
GGIGSDVLR

SEQ ID NO: 43897 - protein, 9 aa, synthetic construct
GGIGSDVVN

SEQ ID NO: 43898 - protein, 9 aa, synthetic construct
GGIGVDTVD

SEQ ID NO: 43899 - protein, 9 aa, synthetic construct
GGIGVDRLV

SEQ ID NO: 43900 - protein, 9 aa, synthetic construct
GGIGVDRMD

SEQ ID NO: 43901 - protein, 9 aa, synthetic construct
GGIGVDRMV

SEQ ID NO: 43902 - protein, 9 aa, synthetic construct
GGIGVDSLN

SEQ ID NO: 43903 - protein, 9 aa, synthetic construct
GGIGVDSLQ

SEQ ID NO: 43904 - protein, 9 aa, synthetic construct
GGIGVDSLS

SEQ ID NO: 43905 - protein, 9 aa, synthetic construct
GGIGVDTAD

SEQ ID NO: 43906 - protein, 9 aa, synthetic construct
GGIGVDTAL

SEQ ID NO: 43907 - protein, 9 aa, synthetic construct
GGIGVDTID

SEQ ID NO: 43908 - protein, 9 aa, synthetic construct
GGIGVDTIE

SEQ ID NO: 43909 - protein, 9 aa, synthetic construct
GGIGVDTLD

SEQ ID NO: 43910 - protein, 9 aa, synthetic construct
GGIGVDTLE

SEQ ID NO: 43911 - protein, 9 aa, synthetic construct
GGIGVDTME

SEQ ID NO: 43912 - protein, 9 aa, synthetic construct
GGIGVDTVS

SEQ ID NO: 43913 - protein, 9 aa, synthetic construct
GGIGVDQLD

SEQ ID NO: 43914 - protein, 9 aa, synthetic construct
GGIGVDTYV

SEQ ID NO: 43915 - protein, 9 aa, synthetic construct
GGIGVDVAR

SEQ ID NO: 43916 - protein, 9 aa, synthetic construct
GGIGVDWAI

SEQ ID NO: 43917 - protein, 9 aa, synthetic construct
GGIGWDDLS

SEQ ID NO: 43918 - protein, 9 aa, synthetic construct
GGIGWDTLD

SEQ ID NO: 43919 - protein, 9 aa, synthetic construct
GGIGWDTMA

SEQ ID NO: 43920 - protein, 9 aa, synthetic construct
GGIGWDTMF

SEQ ID NO: 43921 - protein, 9 aa, synthetic construct
GGIGYDEIL

SEQ ID NO: 43922 - protein, 9 aa, synthetic construct
GGIGYDTLR

SEQ ID NO: 43923 - protein, 9 aa, synthetic construct
GGKGADAID

SEQ ID NO: 43924 - protein, 9 aa, synthetic construct
GGKGADALA

SEQ ID NO: 43925 - protein, 9 aa, synthetic construct
GGKGADALD

SEQ ID NO: 43926 - protein, 9 aa, synthetic construct
GGKGADALN

SEQ ID NO: 43927 - protein, 9 aa, synthetic construct
GGIGVDQVF

SEQ ID NO: 43928 - protein, 9 aa, synthetic construct
GGIGVDLVL

SEQ ID NO: 43929 - protein, 9 aa, synthetic construct
GGIGSDYIE

SEQ ID NO: 43930 - protein, 9 aa, synthetic construct
GGIGTDSLL

SEQ ID NO: 43931 - protein, 9 aa, synthetic construct
GGIGSDYLD

SEQ ID NO: 43932 - protein, 9 aa, synthetic construct
GGIGTDAIY

SEQ ID NO: 43933 - protein, 9 aa, synthetic construct
GGIGTDALH

SEQ ID NO: 43934 - protein, 9 aa, synthetic construct
GGIGTDELI

SEQ ID NO: 43935 - protein, 9 aa, synthetic construct
GGIGTDFLH

SEQ ID NO: 43936 - protein, 9 aa, synthetic construct
GGIGTDKMA

SEQ ID NO: 43937 - protein, 9 aa, synthetic construct
GGIGTDLIE

SEQ ID NO: 43938 - protein, 9 aa, synthetic construct
GGIGTDLVD

SEQ ID NO: 43939 - protein, 9 aa, synthetic construct
GGIGTDMLR

SEQ ID NO: 43940 - protein, 9 aa, synthetic construct
GGIGTDQLF

SEQ ID NO: 43941 - protein, 9 aa, synthetic construct
GGIGTDRLT

SEQ ID NO: 43942 - protein, 9 aa, synthetic construct
GGIGTDRYV

SEQ ID NO: 43943 - protein, 9 aa, synthetic construct
GGIGTDSLA

SEQ ID NO: 43944 - protein, 9 aa, synthetic construct
GGIGTDSMT

SEQ ID NO: 43945 - protein, 9 aa, synthetic construct
GGIGVDLLY

SEQ ID NO: 43946 - protein, 9 aa, synthetic construct
GGIGTDTAE

SEQ ID NO: 43947 - protein, 9 aa, synthetic construct
GGIGTDTAN

SEQ ID NO: 43948 - protein, 9 aa, synthetic construct
GGIGTDTAS

SEQ ID NO: 43949 - protein, 9 aa, synthetic construct
GGIGTDTFV

SEQ ID NO: 43950 - protein, 9 aa, synthetic construct
GGIGTDTLA

SEQ ID NO: 43951 - protein, 9 aa, synthetic construct
GGIGTDTLK

SEQ ID NO: 43952 - protein, 9 aa, synthetic construct
GGIGTDTLV

SEQ ID NO: 43953 - protein, 9 aa, synthetic construct
GGIGTDVLE

SEQ ID NO: 43954 - protein, 9 aa, synthetic construct
GGIGTDVMD

SEQ ID NO: 43955 - protein, 9 aa, synthetic construct
GGIGTDVMQ

SEQ ID NO: 43956 - protein, 9 aa, synthetic construct
GGIGTDVMV

SEQ ID NO: 43957 - protein, 9 aa, synthetic construct
GGIGVDIAD

SEQ ID NO: 43958 - protein, 9 aa, synthetic construct
GGIGVDLIK

SEQ ID NO: 43959 - protein, 9 aa, synthetic construct
GGIGMDVAV

SEQ ID NO: 43960 - protein, 9 aa, synthetic construct
GGIGMDMIW

SEQ ID NO: 43961 - protein, 9 aa, synthetic construct
GGIGMDLLE

SEQ ID NO: 43962 - protein, 9 aa, synthetic construct
GGIGADTYI

SEQ ID NO: 43963 - protein, 9 aa, synthetic construct
GGIGADSIS

SEQ ID NO: 43964 - protein, 9 aa, synthetic construct
GGIGADSIV

SEQ ID NO: 43965 - protein, 9 aa, synthetic construct
GGIGADSIY

SEQ ID NO: 43966 - protein, 9 aa, synthetic construct
GGIGADSLN

SEQ ID NO: 43967 - protein, 9 aa, synthetic construct
GGIGADSLS

SEQ ID NO: 43968 - protein, 9 aa, synthetic construct
GGIGADSMD

SEQ ID NO: 43969 - protein, 9 aa, synthetic construct
GGIGADSME

SEQ ID NO: 43970 - protein, 9 aa, synthetic construct
GGIGADSMH

SEQ ID NO: 43971 - protein, 9 aa, synthetic construct
GGIGADSML

SEQ ID NO: 43972 - protein, 9 aa, synthetic construct
GGIGADSMV

SEQ ID NO: 43973 - protein, 9 aa, synthetic construct
GGIGADSVR

SEQ ID NO: 43974 - protein, 9 aa, synthetic construct
GGIGADSVV

SEQ ID NO: 43975 - protein, 9 aa, synthetic construct
GGIGADSVY

SEQ ID NO: 43976 - protein, 9 aa, synthetic construct
GGIGADTAF

SEQ ID NO: 43977 - protein, 9 aa, synthetic construct
GGIGADTAV

SEQ ID NO: 43978 - protein, 9 aa, synthetic construct
GGIGADTFA

SEQ ID NO: 43979 - protein, 9 aa, synthetic construct
GGIGADTFT

SEQ ID NO: 43980 - protein, 9 aa, synthetic construct
GGIGADTFY

SEQ ID NO: 43981 - protein, 9 aa, synthetic construct
GGIGADTIR

SEQ ID NO: 43982 - protein, 9 aa, synthetic construct
GGIGADTIS

SEQ ID NO: 43983 - protein, 9 aa, synthetic construct
GGIGADTIY

SEQ ID NO: 43984 - protein, 9 aa, synthetic construct
GGIGADTLE

SEQ ID NO: 43985 - protein, 9 aa, synthetic construct
GGIGADTLG

SEQ ID NO: 43986 - protein, 9 aa, synthetic construct
GGIGADTLH

SEQ ID NO: 43987 - protein, 9 aa, synthetic construct
GGIGADTLM

SEQ ID NO: 43988 - protein, 9 aa, synthetic construct
GGIGADTMA

SEQ ID NO: 43989 - protein, 9 aa, synthetic construct
GGIGADTMD

SEQ ID NO: 43990 - protein, 9 aa, synthetic construct
GGIGADTML

SEQ ID NO: 43991 - protein, 9 aa, synthetic construct
GGIGADTVN

SEQ ID NO: 43992 - protein, 9 aa, synthetic construct
GGIGADSIN

SEQ ID NO: 43993 - protein, 9 aa, synthetic construct
GGIGADSII

SEQ ID NO: 43994 - protein, 9 aa, synthetic construct
GGIGADSIF

SEQ ID NO: 43995 - protein, 9 aa, synthetic construct
GGIGADQIY

SEQ ID NO: 43996 - protein, 9 aa, synthetic construct
GGIGADLMH

SEQ ID NO: 43997 - protein, 9 aa, synthetic construct
GGIGADMFD

SEQ ID NO: 43998 - protein, 9 aa, synthetic construct
GGIGADMFV

SEQ ID NO: 43999 - protein, 9 aa, synthetic construct
GGIGADMLF

SEQ ID NO: 44000 - protein, 9 aa, synthetic construct
GGIGADMLH

SEQ ID NO: 44001 - protein, 9 aa, synthetic construct
GGIGADMLI

SEQ ID NO: 44002 - protein, 9 aa, synthetic construct
GGIGADMLL

SEQ ID NO: 44003 - protein, 9 aa, synthetic construct
GGIGADMLN

SEQ ID NO: 44004 - protein, 9 aa, synthetic construct
GGIGADNIK

SEQ ID NO: 44005 - protein, 9 aa, synthetic construct
GGIGADNMT

SEQ ID NO: 44006 - protein, 9 aa, synthetic construct
GGIGADNVK

SEQ ID NO: 44007 - protein, 9 aa, synthetic construct
GGIGADQFF

SEQ ID NO: 44008 - protein, 9 aa, synthetic construct
GGIGADQFL

SEQ ID NO: 44009 - protein, 9 aa, synthetic construct
GGIGADQLA

SEQ ID NO: 44010 - protein, 9 aa, synthetic construct
GGIGADSFV

SEQ ID NO: 44011 - protein, 9 aa, synthetic construct
GGIGADQLF

SEQ ID NO: 44012 - protein, 9 aa, synthetic construct
GGIGADQLW

SEQ ID NO: 44013 - protein, 9 aa, synthetic construct
GGIGADQMR

SEQ ID NO: 44014 - protein, 9 aa, synthetic construct
GGIGADRFK

SEQ ID NO: 44015 - protein, 9 aa, synthetic construct
GGIGADRLK

SEQ ID NO: 44016 - protein, 9 aa, synthetic construct
GGIGADRLL

SEQ ID NO: 44017 - protein, 9 aa, synthetic construct
GGIGADRLN

SEQ ID NO: 44018 - protein, 9 aa, synthetic construct
GGIGADRLS

SEQ ID NO: 44019 - protein, 9 aa, synthetic construct
GGIGADRMI

SEQ ID NO: 44020 - protein, 9 aa, synthetic construct
GGIGADRMS

SEQ ID NO: 44021 - protein, 9 aa, synthetic construct
GGIGADRMT

SEQ ID NO: 44022 - protein, 9 aa, synthetic construct
GGIGADRVF

SEQ ID NO: 44023 - protein, 9 aa, synthetic construct
GGIGADSFH

SEQ ID NO: 44024 - protein, 9 aa, synthetic construct
GGIGADTVS

SEQ ID NO: 44025 - protein, 9 aa, synthetic construct
GGIGADTYY

SEQ ID NO: 44026 - protein, 9 aa, synthetic construct
GGIGLDVLM

SEQ ID NO: 44027 - protein, 9 aa, synthetic construct
GGIGADVIA

SEQ ID NO: 44028 - protein, 9 aa, synthetic construct
GGIGDDELS

SEQ ID NO: 44029 - protein, 9 aa, synthetic construct
GGIGDDEMF

SEQ ID NO: 44030 - protein, 9 aa, synthetic construct
GGIGDDEMW

SEQ ID NO: 44031 - protein, 9 aa, synthetic construct
GGIGDDFID

SEQ ID NO: 44032 - protein, 9 aa, synthetic construct
GGIGDDFIN

SEQ ID NO: 44033 - protein, 9 aa, synthetic construct
GGIGDDFIS

SEQ ID NO: 44034 - protein, 9 aa, synthetic construct
GGIGDDFIT

SEQ ID NO: 44035 - protein, 9 aa, synthetic construct
GGIGDDFIY

SEQ ID NO: 44036 - protein, 9 aa, synthetic construct
GGIGDDFLA

SEQ ID NO: 44037 - protein, 9 aa, synthetic construct
GGIGDDFLD

SEQ ID NO: 44038 - protein, 9 aa, synthetic construct
GGIGDDFLE

SEQ ID NO: 44039 - protein, 9 aa, synthetic construct
GGIGDDFLF

SEQ ID NO: 44040 - protein, 9 aa, synthetic construct
GGIGDDFLH

SEQ ID NO: 44041 - protein, 9 aa, synthetic construct
GGIGDDFLN

SEQ ID NO: 44042 - protein, 9 aa, synthetic construct
GGIGDDFLQ

SEQ ID NO: 44043 - protein, 9 aa, synthetic construct
GGIGDDFLR

SEQ ID NO: 44044 - protein, 9 aa, synthetic construct
GGIGDDFVM

SEQ ID NO: 44045 - protein, 9 aa, synthetic construct
GGIGDDGLF

SEQ ID NO: 44046 - protein, 9 aa, synthetic construct
GGIGDDGLI

SEQ ID NO: 44047 - protein, 9 aa, synthetic construct
GGIGDDGYT

SEQ ID NO: 44048 - protein, 9 aa, synthetic construct
GGIGDDIAV

SEQ ID NO: 44049 - protein, 9 aa, synthetic construct
GGIGDDIFT

SEQ ID NO: 44050 - protein, 9 aa, synthetic construct
GGIGDDIIQ

SEQ ID NO: 44051 - protein, 9 aa, synthetic construct
GGIGDDILG

SEQ ID NO: 44052 - protein, 9 aa, synthetic construct
GGIGDDIML

SEQ ID NO: 44053 - protein, 9 aa, synthetic construct
GGIGDDIMS

SEQ ID NO: 44054 - protein, 9 aa, synthetic construct
GGIGDDIMV

SEQ ID NO: 44055 - protein, 9 aa, synthetic construct
GGIGDDIVF

SEQ ID NO: 44056 - protein, 9 aa, synthetic construct
GGIGDDIVN

SEQ ID NO: 44057 - protein, 9 aa, synthetic construct
GGIGDDELF

SEQ ID NO: 44058 - protein, 9 aa, synthetic construct
GGIGDDDYV

SEQ ID NO: 44059 - protein, 9 aa, synthetic construct
GGIGDDDMD

SEQ ID NO: 44060 - protein, 9 aa, synthetic construct
GGIGADWLT

SEQ ID NO: 44061 - protein, 9 aa, synthetic construct
GGIGADVIK

SEQ ID NO: 44062 - protein, 9 aa, synthetic construct
GGIGADVIL

SEQ ID NO: 44063 - protein, 9 aa, synthetic construct
GGIGADVIM

SEQ ID NO: 44064 - protein, 9 aa, synthetic construct
GGIGADVIY

SEQ ID NO: 44065 - protein, 9 aa, synthetic construct
GGIGADVLL

SEQ ID NO: 44066 - protein, 9 aa, synthetic construct
GGIGADVLV

SEQ ID NO: 44067 - protein, 9 aa, synthetic construct
GGIGADVMD

SEQ ID NO: 44068 - protein, 9 aa, synthetic construct
GGIGADVMI

SEQ ID NO: 44069 - protein, 9 aa, synthetic construct
GGIGADVML

SEQ ID NO: 44070 - protein, 9 aa, synthetic construct
GGIGADVMV

SEQ ID NO: 44071 - protein, 9 aa, synthetic construct
GGIGADVVD

SEQ ID NO: 44072 - protein, 9 aa, synthetic construct
GGIGADWLD

SEQ ID NO: 44073 - protein, 9 aa, synthetic construct
GGIGADWLR

SEQ ID NO: 44074 - protein, 9 aa, synthetic construct
GGIGADYID

SEQ ID NO: 44075 - protein, 9 aa, synthetic construct
GGIGDDDLW

SEQ ID NO: 44076 - protein, 9 aa, synthetic construct
GGIGADYLA

SEQ ID NO: 44077 - protein, 9 aa, synthetic construct
GGIGADYLD

SEQ ID NO: 44078 - protein, 9 aa, synthetic construct
GGIGADYLW

SEQ ID NO: 44079 - protein, 9 aa, synthetic construct
GGIGADYLY

SEQ ID NO: 44080 - protein, 9 aa, synthetic construct
GGIGADYMS

SEQ ID NO: 44081 - protein, 9 aa, synthetic construct
GGIGADYMY

SEQ ID NO: 44082 - protein, 9 aa, synthetic construct
GGIGDDALD

SEQ ID NO: 44083 - protein, 9 aa, synthetic construct
GGIGDDALR

SEQ ID NO: 44084 - protein, 9 aa, synthetic construct
GGIGDDALW

SEQ ID NO: 44085 - protein, 9 aa, synthetic construct
GGIGDDAVS

SEQ ID NO: 44086 - protein, 9 aa, synthetic construct
GGIGDDDLA

SEQ ID NO: 44087 - protein, 9 aa, synthetic construct
GGIGDDDLF

SEQ ID NO: 44088 - protein, 9 aa, synthetic construct
GGIGDDDLK

SEQ ID NO: 44089 - protein, 9 aa, synthetic construct
GGIGADLMD

SEQ ID NO: 44090 - protein, 9 aa, synthetic construct
GGIGADLLQ

SEQ ID NO: 44091 - protein, 9 aa, synthetic construct
GGIGADLLM

SEQ ID NO: 44092 - protein, 9 aa, synthetic construct
GGIGADLLL

SEQ ID NO: 44093 - protein, 9 aa, synthetic construct
GGHGRDTLI

SEQ ID NO: 44094 - protein, 9 aa, synthetic construct
GGHGRDTLK

SEQ ID NO: 44095 - protein, 9 aa, synthetic construct
GGHGRDTLN

SEQ ID NO: 44096 - protein, 9 aa, synthetic construct
GGHGRDTLT

SEQ ID NO: 44097 - protein, 9 aa, synthetic construct
GGHGRDVFI

SEQ ID NO: 44098 - protein, 9 aa, synthetic construct
GGHGRDVID

SEQ ID NO: 44099 - protein, 9 aa, synthetic construct
GGHGRDVLL

SEQ ID NO: 44100 - protein, 9 aa, synthetic construct
GGHGSDEID

SEQ ID NO: 44101 - protein, 9 aa, synthetic construct
GGHGSDELF

SEQ ID NO: 44102 - protein, 9 aa, synthetic construct
GGHGSDELH

SEQ ID NO: 44103 - protein, 9 aa, synthetic construct
GGHGSDELR

SEQ ID NO: 44104 - protein, 9 aa, synthetic construct
GGHGSDHLD

SEQ ID NO: 44105 - protein, 9 aa, synthetic construct
GGHGSDILL

SEQ ID NO: 44106 - protein, 9 aa, synthetic construct
GGHGSDLLI

SEQ ID NO: 44107 - protein, 9 aa, synthetic construct
GGHGSDMIA

SEQ ID NO: 44108 - protein, 9 aa, synthetic construct
GGHGSDMLF

SEQ ID NO: 44109 - protein, 9 aa, synthetic construct
GGHGSDQLR

SEQ ID NO: 44110 - protein, 9 aa, synthetic construct
GGHGSDRAT

SEQ ID NO: 44111 - protein, 9 aa, synthetic construct
GGHGSDRIS

SEQ ID NO: 44112 - protein, 9 aa, synthetic construct
GGHGSDSFV

SEQ ID NO: 44113 - protein, 9 aa, synthetic construct
GGHGSDSIL

SEQ ID NO: 44114 - protein, 9 aa, synthetic construct
GGHGSDSIY

SEQ ID NO: 44115 - protein, 9 aa, synthetic construct
GGHGSDTIS

SEQ ID NO: 44116 - protein, 9 aa, synthetic construct
GGHGSDTLN

SEQ ID NO: 44117 - protein, 9 aa, synthetic construct
GGHGSDTLT

SEQ ID NO: 44118 - protein, 9 aa, synthetic construct
GGHGSDTYY

SEQ ID NO: 44119 - protein, 9 aa, synthetic construct
GGHGSDVYR

SEQ ID NO: 44120 - protein, 9 aa, synthetic construct
GGHGSDWLF

SEQ ID NO: 44121 - protein, 9 aa, synthetic construct
GGHGSDYID

SEQ ID NO: 44122 - protein, 9 aa, synthetic construct
GGHGRDRLE

SEQ ID NO: 44123 - protein, 9 aa, synthetic construct
GGHGRDRFE

SEQ ID NO: 44124 - protein, 9 aa, synthetic construct
GGHGRDQIR

SEQ ID NO: 44125 - protein, 9 aa, synthetic construct
GGHGQDLLE

SEQ ID NO: 44126 - protein, 9 aa, synthetic construct
GGHGNDVVT

SEQ ID NO: 44127 - protein, 9 aa, synthetic construct
GGHGNDWLS

SEQ ID NO: 44128 - protein, 9 aa, synthetic construct
GGHGNDWLY

SEQ ID NO: 44129 - protein, 9 aa, synthetic construct
GGHGNDWVL

SEQ ID NO: 44130 - protein, 9 aa, synthetic construct
GGHGNDYLL

SEQ ID NO: 44131 - protein, 9 aa, synthetic construct
GGHGPDALR

SEQ ID NO: 44132 - protein, 9 aa, synthetic construct
GGHGPDKLD

SEQ ID NO: 44133 - protein, 9 aa, synthetic construct
GGHGPDLFV

SEQ ID NO: 44134 - protein, 9 aa, synthetic construct
GGHGPDPLT

SEQ ID NO: 44135 - protein, 9 aa, synthetic construct
GGHGQDEIF

SEQ ID NO: 44136 - protein, 9 aa, synthetic construct
GGHGQDKIR

SEQ ID NO: 44137 - protein, 9 aa, synthetic construct
GGHGQDKLF

SEQ ID NO: 44138 - protein, 9 aa, synthetic construct
GGHGQDLAV

SEQ ID NO: 44139 - protein, 9 aa, synthetic construct
GGHGQDLVS

SEQ ID NO: 44140 - protein, 9 aa, synthetic construct
GGHGRDQID

SEQ ID NO: 44141 - protein, 9 aa, synthetic construct
GGHGQDMLH

SEQ ID NO: 44142 - protein, 9 aa, synthetic construct
GGHGQDQIE

SEQ ID NO: 44143 - protein, 9 aa, synthetic construct
GGHGQDRML

SEQ ID NO: 44144 - protein, 9 aa, synthetic construct
GGHGQDSLT

SEQ ID NO: 44145 - protein, 9 aa, synthetic construct
GGHGQDTLI

SEQ ID NO: 44146 - protein, 9 aa, synthetic construct
GGHGQDTLN

SEQ ID NO: 44147 - protein, 9 aa, synthetic construct
GGHGQDTLV

SEQ ID NO: 44148 - protein, 9 aa, synthetic construct
GGHGRDALY

SEQ ID NO: 44149 - protein, 9 aa, synthetic construct
GGHGRDDIA

SEQ ID NO: 44150 - protein, 9 aa, synthetic construct
GGHGRDGIY

SEQ ID NO: 44151 - protein, 9 aa, synthetic construct
GGHGRDLLF

SEQ ID NO: 44152 - protein, 9 aa, synthetic construct
GGHGRDLLI

SEQ ID NO: 44153 - protein, 9 aa, synthetic construct
GGHGRDLLR

SEQ ID NO: 44154 - protein, 9 aa, synthetic construct
GGHGSDYVD

SEQ ID NO: 44155 - protein, 9 aa, synthetic construct
GGHGTDELY

SEQ ID NO: 44156 - protein, 9 aa, synthetic construct
GGHGTDILI

SEQ ID NO: 44157 - protein, 9 aa, synthetic construct
GGIGADKIL

SEQ ID NO: 44158 - protein, 9 aa, synthetic construct
GGIGADELH

SEQ ID NO: 44159 - protein, 9 aa, synthetic construct
GGIGADELL

SEQ ID NO: 44160 - protein, 9 aa, synthetic construct
GGIGADELQ

SEQ ID NO: 44161 - protein, 9 aa, synthetic construct
GGIGADELR

SEQ ID NO: 44162 - protein, 9 aa, synthetic construct
GGIGADFID

SEQ ID NO: 44163 - protein, 9 aa, synthetic construct
GGIGADFLE

SEQ ID NO: 44164 - protein, 9 aa, synthetic construct
GGIGADGLD

SEQ ID NO: 44165 - protein, 9 aa, synthetic construct
GGIGADHLV

SEQ ID NO: 44166 - protein, 9 aa, synthetic construct
GGIGADILD

SEQ ID NO: 44167 - protein, 9 aa, synthetic construct
GGIGADILF

SEQ ID NO: 44168 - protein, 9 aa, synthetic construct
GGIGADILH

SEQ ID NO: 44169 - protein, 9 aa, synthetic construct
GGIGADILL

SEQ ID NO: 44170 - protein, 9 aa, synthetic construct
GGIGADILS

SEQ ID NO: 44171 - protein, 9 aa, synthetic construct
GGIGADKLL

SEQ ID NO: 44172 - protein, 9 aa, synthetic construct
GGIGADELD

SEQ ID NO: 44173 - protein, 9 aa, synthetic construct
GGIGADKLS

SEQ ID NO: 44174 - protein, 9 aa, synthetic construct
GGIGADKLV

SEQ ID NO: 44175 - protein, 9 aa, synthetic construct
GGIGADKMF

SEQ ID NO: 44176 - protein, 9 aa, synthetic construct
GGIGADKMT

SEQ ID NO: 44177 - protein, 9 aa, synthetic construct
GGIGADLIF

SEQ ID NO: 44178 - protein, 9 aa, synthetic construct
GGIGADLIK

SEQ ID NO: 44179 - protein, 9 aa, synthetic construct
GGIGADLIN

SEQ ID NO: 44180 - protein, 9 aa, synthetic construct
GGIGADLIS

SEQ ID NO: 44181 - protein, 9 aa, synthetic construct
GGIGADLIT

SEQ ID NO: 44182 - protein, 9 aa, synthetic construct
GGIGADLLA

SEQ ID NO: 44183 - protein, 9 aa, synthetic construct
GGIGADLLE

SEQ ID NO: 44184 - protein, 9 aa, synthetic construct
GGIGADLLH

SEQ ID NO: 44185 - protein, 9 aa, synthetic construct
GGIGADLLK

SEQ ID NO: 44186 - protein, 9 aa, synthetic construct
GGIGADELF

SEQ ID NO: 44187 - protein, 9 aa, synthetic construct
GGIGADEID

SEQ ID NO: 44188 - protein, 9 aa, synthetic construct
GGHGTDLIS

SEQ ID NO: 44189 - protein, 9 aa, synthetic construct
GGHGYDILD

SEQ ID NO: 44190 - protein, 9 aa, synthetic construct
GGHGTDSLS

SEQ ID NO: 44191 - protein, 9 aa, synthetic construct
GGHGTDTAT

SEQ ID NO: 44192 - protein, 9 aa, synthetic construct
GGHGTDTLD

SEQ ID NO: 44193 - protein, 9 aa, synthetic construct
GGHGTDTLI

SEQ ID NO: 44194 - protein, 9 aa, synthetic construct
GGHGTDTLY

SEQ ID NO: 44195 - protein, 9 aa, synthetic construct
GGHGVDELL

SEQ ID NO: 44196 - protein, 9 aa, synthetic construct
GGHGVDFID

SEQ ID NO: 44197 - protein, 9 aa, synthetic construct
GGHGVDLII

SEQ ID NO: 44198 - protein, 9 aa, synthetic construct
GGHGVDLLF

SEQ ID NO: 44199 - protein, 9 aa, synthetic construct
GGHGVDQLF

SEQ ID NO: 44200 - protein, 9 aa, synthetic construct
GGHGVDTLF

SEQ ID NO: 44201 - protein, 9 aa, synthetic construct
GGHGVDYLD

SEQ ID NO: 44202 - protein, 9 aa, synthetic construct
GGHGWDKLF

SEQ ID NO: 44203 - protein, 9 aa, synthetic construct
GGHGYDRLS

SEQ ID NO: 44204 - protein, 9 aa, synthetic construct
GGIGADDMV

SEQ ID NO: 44205 - protein, 9 aa, synthetic construct
GGHGYDVLV

SEQ ID NO: 44206 - protein, 9 aa, synthetic construct
GGIGADALD

SEQ ID NO: 44207 - protein, 9 aa, synthetic construct
GGIGADALN

SEQ ID NO: 44208 - protein, 9 aa, synthetic construct
GGIGADALT

SEQ ID NO: 44209 - protein, 9 aa, synthetic construct
GGIGADAMA

SEQ ID NO: 44210 - protein, 9 aa, synthetic construct
GGIGADAMN

SEQ ID NO: 44211 - protein, 9 aa, synthetic construct
GGIGADAMS

SEQ ID NO: 44212 - protein, 9 aa, synthetic construct
GGIGADAMY

SEQ ID NO: 44213 - protein, 9 aa, synthetic construct
GGIGADDFI

SEQ ID NO: 44214 - protein, 9 aa, synthetic construct
GGIGADDIS

SEQ ID NO: 44215 - protein, 9 aa, synthetic construct
GGIGADDLA

SEQ ID NO: 44216 - protein, 9 aa, synthetic construct
GGIGADDLR

SEQ ID NO: 44217 - protein, 9 aa, synthetic construct
GGIGADDLS

SEQ ID NO: 44218 - protein, 9 aa, synthetic construct
GGIGDDIVV

SEQ ID NO: 44219 - protein, 9 aa, synthetic construct
GGIGDDIYI

SEQ ID NO: 44220 - protein, 9 aa, synthetic construct
GGIGDDKIE

SEQ ID NO: 44221 - protein, 9 aa, synthetic construct
GGIGGDILT

SEQ ID NO: 44222 - protein, 9 aa, synthetic construct
GGIGHDLLR

SEQ ID NO: 44223 - protein, 9 aa, synthetic construct
GGIGHDLLS

SEQ ID NO: 44224 - protein, 9 aa, synthetic construct
GGIGHDLLV

SEQ ID NO: 44225 - protein, 9 aa, synthetic construct
GGIGHDLMA

SEQ ID NO: 44226 - protein, 9 aa, synthetic construct
GGIGHDMLQ

SEQ ID NO: 44227 - protein, 9 aa, synthetic construct
GGIGHDNLS

SEQ ID NO: 44228 - protein, 9 aa, synthetic construct
GGIGHDQID

SEQ ID NO: 44229 - protein, 9 aa, synthetic construct
GGIGHDQLV

SEQ ID NO: 44230 - protein, 9 aa, synthetic construct
GGIGHDRLD

SEQ ID NO: 44231 - protein, 9 aa, synthetic construct
GGIGHDRLE

SEQ ID NO: 44232 - protein, 9 aa, synthetic construct
GGIGHDRLH

SEQ ID NO: 44233 - protein, 9 aa, synthetic construct
GGIGHDRLI

SEQ ID NO: 44234 - protein, 9 aa, synthetic construct
GGIGHDSIF

SEQ ID NO: 44235 - protein, 9 aa, synthetic construct
GGIGHDSLW

SEQ ID NO: 44236 - protein, 9 aa, synthetic construct
GGIGHDTIS

SEQ ID NO: 44237 - protein, 9 aa, synthetic construct
GGIGHDTIT

SEQ ID NO: 44238 - protein, 9 aa, synthetic construct
GGIGHDTIV

SEQ ID NO: 44239 - protein, 9 aa, synthetic construct
GGIGHDTLF

SEQ ID NO: 44240 - protein, 9 aa, synthetic construct
GGIGHDTLH

SEQ ID NO: 44241 - protein, 9 aa, synthetic construct
GGIGHDTLT

SEQ ID NO: 44242 - protein, 9 aa, synthetic construct
GGIGHDTMR

SEQ ID NO: 44243 - protein, 9 aa, synthetic construct
GGIGHDTVV

SEQ ID NO: 44244 - protein, 9 aa, synthetic construct
GGIGHDVIR

SEQ ID NO: 44245 - protein, 9 aa, synthetic construct
GGIGHDVIT

SEQ ID NO: 44246 - protein, 9 aa, synthetic construct
GGIGHDVLG

SEQ ID NO: 44247 - protein, 9 aa, synthetic construct
GGIGHDVVA

SEQ ID NO: 44248 - protein, 9 aa, synthetic construct
GGIGHDWLA

SEQ ID NO: 44249 - protein, 9 aa, synthetic construct
GGIGHDYLT

SEQ ID NO: 44250 - protein, 9 aa, synthetic construct
GGIGIDAAA

SEQ ID NO: 44251 - protein, 9 aa, synthetic construct
GGIGHDKLK

SEQ ID NO: 44252 - protein, 9 aa, synthetic construct
GGIGHDILT

SEQ ID NO: 44253 - protein, 9 aa, synthetic construct
GGIGHDILL

SEQ ID NO: 44254 - protein, 9 aa, synthetic construct
GGIGGDTLY

SEQ ID NO: 44255 - protein, 9 aa, synthetic construct
GGIGGDLLC

SEQ ID NO: 44256 - protein, 9 aa, synthetic construct
GGIGGDLLW

SEQ ID NO: 44257 - protein, 9 aa, synthetic construct
GGIGGDLMN

SEQ ID NO: 44258 - protein, 9 aa, synthetic construct
GGIGGDQIL

SEQ ID NO: 44259 - protein, 9 aa, synthetic construct
GGIGGDQIR

SEQ ID NO: 44260 - protein, 9 aa, synthetic construct
GGIGGDQLE

SEQ ID NO: 44261 - protein, 9 aa, synthetic construct
GGIGGDRLI

SEQ ID NO: 44262 - protein, 9 aa, synthetic construct
GGIGGDSIF

SEQ ID NO: 44263 - protein, 9 aa, synthetic construct
GGIGGDSIL

SEQ ID NO: 44264 - protein, 9 aa, synthetic construct
GGIGGDTIN

SEQ ID NO: 44265 - protein, 9 aa, synthetic construct
GGIGGDTLK

SEQ ID NO: 44266 - protein, 9 aa, synthetic construct
GGIGGDTLL

SEQ ID NO: 44267 - protein, 9 aa, synthetic construct
GGIGGDTLR

SEQ ID NO: 44268 - protein, 9 aa, synthetic construct
GGIGGDTVF

SEQ ID NO: 44269 - protein, 9 aa, synthetic construct
GGIGHDILI

SEQ ID NO: 44270 - protein, 9 aa, synthetic construct
GGIGGDTYY

SEQ ID NO: 44271 - protein, 9 aa, synthetic construct
GGIGGDVAY

SEQ ID NO: 44272 - protein, 9 aa, synthetic construct
GGIGGDVLI

SEQ ID NO: 44273 - protein, 9 aa, synthetic construct
GGIGGDVLN

SEQ ID NO: 44274 - protein, 9 aa, synthetic construct
GGIGGDVLT

SEQ ID NO: 44275 - protein, 9 aa, synthetic construct
GGIGGDVMH

SEQ ID NO: 44276 - protein, 9 aa, synthetic construct
GGIGHDALH

SEQ ID NO: 44277 - protein, 9 aa, synthetic construct
GGIGHDDLD

SEQ ID NO: 44278 - protein, 9 aa, synthetic construct
GGIGHDDLR

SEQ ID NO: 44279 - protein, 9 aa, synthetic construct
GGIGHDEIN

SEQ ID NO: 44280 - protein, 9 aa, synthetic construct
GGIGHDELQ

SEQ ID NO: 44281 - protein, 9 aa, synthetic construct
GGIGHDFLV

SEQ ID NO: 44282 - protein, 9 aa, synthetic construct
GGIGHDHID

SEQ ID NO: 44283 - protein, 9 aa, synthetic construct
GGIGIDDLQ

SEQ ID NO: 44284 - protein, 9 aa, synthetic construct
GGIGIDELS

SEQ ID NO: 44285 - protein, 9 aa, synthetic construct
GGIGIDFLK

SEQ ID NO: 44286 - protein, 9 aa, synthetic construct
GGIGLDGVK

SEQ ID NO: 44287 - protein, 9 aa, synthetic construct
GGIGKDTIS

SEQ ID NO: 44288 - protein, 9 aa, synthetic construct
GGIGKDTLA

SEQ ID NO: 44289 - protein, 9 aa, synthetic construct
GGIGKDTLE

SEQ ID NO: 44290 - protein, 9 aa, synthetic construct
GGIGKDTLI

SEQ ID NO: 44291 - protein, 9 aa, synthetic construct
GGIGKDTLL

SEQ ID NO: 44292 - protein, 9 aa, synthetic construct
GGIGKDTLR

SEQ ID NO: 44293 - protein, 9 aa, synthetic construct
GGIGKDTLY

SEQ ID NO: 44294 - protein, 9 aa, synthetic construct
GGIGKDVLG

SEQ ID NO: 44295 - protein, 9 aa, synthetic construct
GGIGKDVLH

SEQ ID NO: 44296 - protein, 9 aa, synthetic construct
GGIGKDVLT

SEQ ID NO: 44297 - protein, 9 aa, synthetic construct
GGIGKDWAQ

SEQ ID NO: 44298 - protein, 9 aa, synthetic construct
GGIGKDWLS

SEQ ID NO: 44299 - protein, 9 aa, synthetic construct
GGIGLDDIS

SEQ ID NO: 44300 - protein, 9 aa, synthetic construct
GGIGLDIII

SEQ ID NO: 44301 - protein, 9 aa, synthetic construct
GGIGKDTID

SEQ ID NO: 44302 - protein, 9 aa, synthetic construct
GGIGLDILD

SEQ ID NO: 44303 - protein, 9 aa, synthetic construct
GGIGLDKAL

SEQ ID NO: 44304 - protein, 9 aa, synthetic construct
GGIGLDKLT

SEQ ID NO: 44305 - protein, 9 aa, synthetic construct
GGIGLDLLD

SEQ ID NO: 44306 - protein, 9 aa, synthetic construct
GGIGLDLLR

SEQ ID NO: 44307 - protein, 9 aa, synthetic construct
GGIGLDMLY

SEQ ID NO: 44308 - protein, 9 aa, synthetic construct
GGIGLDSLF

SEQ ID NO: 44309 - protein, 9 aa, synthetic construct
GGIGLDTIY

SEQ ID NO: 44310 - protein, 9 aa, synthetic construct
GGIGLDTLQ

SEQ ID NO: 44311 - protein, 9 aa, synthetic construct
GGIGLDTLY

SEQ ID NO: 44312 - protein, 9 aa, synthetic construct
GGIGLDTMT

SEQ ID NO: 44313 - protein, 9 aa, synthetic construct
GGIGLDTVV

SEQ ID NO: 44314 - protein, 9 aa, synthetic construct
GGIGLDVFL

SEQ ID NO: 44315 - protein, 9 aa, synthetic construct
GGIGKDTIF

SEQ ID NO: 44316 - protein, 9 aa, synthetic construct
GGIGKDSML

SEQ ID NO: 44317 - protein, 9 aa, synthetic construct
GGIGIDFLN

SEQ ID NO: 44318 - protein, 9 aa, synthetic construct
GGIGIDTIW

SEQ ID NO: 44319 - protein, 9 aa, synthetic construct
GGIGIDILD

SEQ ID NO: 44320 - protein, 9 aa, synthetic construct
GGIGIDILS

SEQ ID NO: 44321 - protein, 9 aa, synthetic construct
GGIGIDILV

SEQ ID NO: 44322 - protein, 9 aa, synthetic construct
GGIGIDKIS

SEQ ID NO: 44323 - protein, 9 aa, synthetic construct
GGIGIDKLI

SEQ ID NO: 44324 - protein, 9 aa, synthetic construct
GGIGIDLLF

SEQ ID NO: 44325 - protein, 9 aa, synthetic construct
GGIGIDLLS

SEQ ID NO: 44326 - protein, 9 aa, synthetic construct
GGIGIDQIA

SEQ ID NO: 44327 - protein, 9 aa, synthetic construct
GGIGIDQIW

SEQ ID NO: 44328 - protein, 9 aa, synthetic construct
GGIGIDQLA

SEQ ID NO: 44329 - protein, 9 aa, synthetic construct
GGIGIDRMT

SEQ ID NO: 44330 - protein, 9 aa, synthetic construct
GGIGIDTAD

SEQ ID NO: 44331 - protein, 9 aa, synthetic construct
GGIGIDTAT

SEQ ID NO: 44332 - protein, 9 aa, synthetic construct
GGIGIDTLL

SEQ ID NO: 44333 - protein, 9 aa, synthetic construct
GGIGKDSIN

SEQ ID NO: 44334 - protein, 9 aa, synthetic construct
GGIGIDTYA

SEQ ID NO: 44335 - protein, 9 aa, synthetic construct
GGIGIDVFI

SEQ ID NO: 44336 - protein, 9 aa, synthetic construct
GGIGIDYLD

SEQ ID NO: 44337 - protein, 9 aa, synthetic construct
GGIGKDFLY

SEQ ID NO: 44338 - protein, 9 aa, synthetic construct
GGIGKDGLF

SEQ ID NO: 44339 - protein, 9 aa, synthetic construct
GGIGKDKLF

SEQ ID NO: 44340 - protein, 9 aa, synthetic construct
GGIGKDKYT

SEQ ID NO: 44341 - protein, 9 aa, synthetic construct
GGIGKDLLD

SEQ ID NO: 44342 - protein, 9 aa, synthetic construct
GGIGKDMLH

SEQ ID NO: 44343 - protein, 9 aa, synthetic construct
GGIGKDRLD

SEQ ID NO: 44344 - protein, 9 aa, synthetic construct
GGIGKDRLF

SEQ ID NO: 44345 - protein, 9 aa, synthetic construct
GGIGKDRLT

SEQ ID NO: 44346 - protein, 9 aa, synthetic construct
GGIGKDSFI

SEQ ID NO: 44347 - protein, 9 aa, synthetic construct
GGIGGDIML

SEQ ID NO: 44348 - protein, 9 aa, synthetic construct
GGIGGDILE

SEQ ID NO: 44349 - protein, 9 aa, synthetic construct
GGIGDDKIF

SEQ ID NO: 44350 - protein, 9 aa, synthetic construct
GGIGGDGLY

SEQ ID NO: 44351 - protein, 9 aa, synthetic construct
GGIGDDRFV

SEQ ID NO: 44352 - protein, 9 aa, synthetic construct
GGIGDDRIA

SEQ ID NO: 44353 - protein, 9 aa, synthetic construct
GGIGDDRLA

SEQ ID NO: 44354 - protein, 9 aa, synthetic construct
GGIGDDRLD

SEQ ID NO: 44355 - protein, 9 aa, synthetic construct
GGIGDDRMH

SEQ ID NO: 44356 - protein, 9 aa, synthetic construct
GGIGDDRMY

SEQ ID NO: 44357 - protein, 9 aa, synthetic construct
GGIGDDRVD

SEQ ID NO: 44358 - protein, 9 aa, synthetic construct
GGIGDDSAW

SEQ ID NO: 44359 - protein, 9 aa, synthetic construct
GGIGDDSII

SEQ ID NO: 44360 - protein, 9 aa, synthetic construct
GGIGDDSIV

SEQ ID NO: 44361 - protein, 9 aa, synthetic construct
GGIGDDSLE

SEQ ID NO: 44362 - protein, 9 aa, synthetic construct
GGIGDDSLQ

SEQ ID NO: 44363 - protein, 9 aa, synthetic construct
GGIGDDSLT

SEQ ID NO: 44364 - protein, 9 aa, synthetic construct
GGIGDDSLW

SEQ ID NO: 44365 - protein, 9 aa, synthetic construct
GGIGDDSMD

SEQ ID NO: 44366 - protein, 9 aa, synthetic construct
GGIGDDSVL

SEQ ID NO: 44367 - protein, 9 aa, synthetic construct
GGIGDDSVS

SEQ ID NO: 44368 - protein, 9 aa, synthetic construct
GGIGDDSYF

SEQ ID NO: 44369 - protein, 9 aa, synthetic construct
GGIGDDTAF

SEQ ID NO: 44370 - protein, 9 aa, synthetic construct
GGIGDDTFE

SEQ ID NO: 44371 - protein, 9 aa, synthetic construct
GGIGDDTFL

SEQ ID NO: 44372 - protein, 9 aa, synthetic construct
GGIGDDTIA

SEQ ID NO: 44373 - protein, 9 aa, synthetic construct
GGIGDDTIE

SEQ ID NO: 44374 - protein, 9 aa, synthetic construct
GGIGDDTIG

SEQ ID NO: 44375 - protein, 9 aa, synthetic construct
GGIGDDTII

SEQ ID NO: 44376 - protein, 9 aa, synthetic construct
GGIGDDTIQ

SEQ ID NO: 44377 - protein, 9 aa, synthetic construct
GGIGDDTIS

SEQ ID NO: 44378 - protein, 9 aa, synthetic construct
GGIGDDTIT

SEQ ID NO: 44379 - protein, 9 aa, synthetic construct
GGIGDDTLQ

SEQ ID NO: 44380 - protein, 9 aa, synthetic construct
GGIGDDQVN

SEQ ID NO: 44381 - protein, 9 aa, synthetic construct
GGIGDDQLQ

SEQ ID NO: 44382 - protein, 9 aa, synthetic construct
GGIGDDQLK

SEQ ID NO: 44383 - protein, 9 aa, synthetic construct
GGIGDDLLM

SEQ ID NO: 44384 - protein, 9 aa, synthetic construct
GGIGDDKLG

SEQ ID NO: 44385 - protein, 9 aa, synthetic construct
GGIGDDKLS

SEQ ID NO: 44386 - protein, 9 aa, synthetic construct
GGIGDDKVE

SEQ ID NO: 44387 - protein, 9 aa, synthetic construct
GGIGDDLIE

SEQ ID NO: 44388 - protein, 9 aa, synthetic construct
GGIGDDLIK

SEQ ID NO: 44389 - protein, 9 aa, synthetic construct
GGIGDDLIL

SEQ ID NO: 44390 - protein, 9 aa, synthetic construct
GGIGDDLIS

SEQ ID NO: 44391 - protein, 9 aa, synthetic construct
GGIGDDLIV

SEQ ID NO: 44392 - protein, 9 aa, synthetic construct
GGIGDDLLF

SEQ ID NO: 44393 - protein, 9 aa, synthetic construct
GGIGDDLLG

SEQ ID NO: 44394 - protein, 9 aa, synthetic construct
GGIGDDLLI

SEQ ID NO: 44395 - protein, 9 aa, synthetic construct
GGIGDDLLK

SEQ ID NO: 44396 - protein, 9 aa, synthetic construct
GGIGDDLLL

SEQ ID NO: 44397 - protein, 9 aa, synthetic construct
GGIGDDLLS

SEQ ID NO: 44398 - protein, 9 aa, synthetic construct
GGIGDDQLH

SEQ ID NO: 44399 - protein, 9 aa, synthetic construct
GGIGDDLMI

SEQ ID NO: 44400 - protein, 9 aa, synthetic construct
GGIGDDLMY

SEQ ID NO: 44401 - protein, 9 aa, synthetic construct
GGIGDDLVI

SEQ ID NO: 44402 - protein, 9 aa, synthetic construct
GGIGDDLYH

SEQ ID NO: 44403 - protein, 9 aa, synthetic construct
GGIGDDLYY

SEQ ID NO: 44404 - protein, 9 aa, synthetic construct
GGIGDDMIN

SEQ ID NO: 44405 - protein, 9 aa, synthetic construct
GGIGDDMLN

SEQ ID NO: 44406 - protein, 9 aa, synthetic construct
GGIGDDMLS

SEQ ID NO: 44407 - protein, 9 aa, synthetic construct
GGIGDDNYH

SEQ ID NO: 44408 - protein, 9 aa, synthetic construct
GGIGDDQII

SEQ ID NO: 44409 - protein, 9 aa, synthetic construct
GGIGDDQIY

SEQ ID NO: 44410 - protein, 9 aa, synthetic construct
GGIGDDQLD

SEQ ID NO: 44411 - protein, 9 aa, synthetic construct
GGIGDDQLE

SEQ ID NO: 44412 - protein, 9 aa, synthetic construct
GGIGDDTMN

SEQ ID NO: 44413 - protein, 9 aa, synthetic construct
GGIGDDTMR

SEQ ID NO: 44414 - protein, 9 aa, synthetic construct
GGIGDDTMY

SEQ ID NO: 44415 - protein, 9 aa, synthetic construct
GGIGFDDLT

SEQ ID NO: 44416 - protein, 9 aa, synthetic construct
GGIGEDSLS

SEQ ID NO: 44417 - protein, 9 aa, synthetic construct
GGIGEDTFR

SEQ ID NO: 44418 - protein, 9 aa, synthetic construct
GGIGEDTLA

SEQ ID NO: 44419 - protein, 9 aa, synthetic construct
GGIGEDTLD

SEQ ID NO: 44420 - protein, 9 aa, synthetic construct
GGIGEDTLI

SEQ ID NO: 44421 - protein, 9 aa, synthetic construct
GGIGEDTMI

SEQ ID NO: 44422 - protein, 9 aa, synthetic construct
GGIGEDTVR

SEQ ID NO: 44423 - protein, 9 aa, synthetic construct
GGIGEDTYI

SEQ ID NO: 44424 - protein, 9 aa, synthetic construct
GGIGEDVFS

SEQ ID NO: 44425 - protein, 9 aa, synthetic construct
GGIGEDVLY

SEQ ID NO: 44426 - protein, 9 aa, synthetic construct
GGIGEDVMT

SEQ ID NO: 44427 - protein, 9 aa, synthetic construct
GGIGEDWLY

SEQ ID NO: 44428 - protein, 9 aa, synthetic construct
GGIGEDYLY

SEQ ID NO: 44429 - protein, 9 aa, synthetic construct
GGIGFDEVF

SEQ ID NO: 44430 - protein, 9 aa, synthetic construct
GGIGEDNYY

SEQ ID NO: 44431 - protein, 9 aa, synthetic construct
GGIGFDMLN

SEQ ID NO: 44432 - protein, 9 aa, synthetic construct
GGIGFDMLT

SEQ ID NO: 44433 - protein, 9 aa, synthetic construct
GGIGFDSLM

SEQ ID NO: 44434 - protein, 9 aa, synthetic construct
GGIGFDSME

SEQ ID NO: 44435 - protein, 9 aa, synthetic construct
GGIGFDTIE

SEQ ID NO: 44436 - protein, 9 aa, synthetic construct
GGIGFDTIN

SEQ ID NO: 44437 - protein, 9 aa, synthetic construct
GGIGFDTIR

SEQ ID NO: 44438 - protein, 9 aa, synthetic construct
GGIGFDTIT

SEQ ID NO: 44439 - protein, 9 aa, synthetic construct
GGIGFDTLN

SEQ ID NO: 44440 - protein, 9 aa, synthetic construct
GGIGFDVVS

SEQ ID NO: 44441 - protein, 9 aa, synthetic construct
GGIGGDDLD

SEQ ID NO: 44442 - protein, 9 aa, synthetic construct
GGIGGDELD

SEQ ID NO: 44443 - protein, 9 aa, synthetic construct
GGIGGDELY

SEQ ID NO: 44444 - protein, 9 aa, synthetic construct
GGIGEDRLI

SEQ ID NO: 44445 - protein, 9 aa, synthetic construct
GGIGEDLLT

SEQ ID NO: 44446 - protein, 9 aa, synthetic construct
GGIGDDTVA

SEQ ID NO: 44447 - protein, 9 aa, synthetic construct
GGIGDDVYY

SEQ ID NO: 44448 - protein, 9 aa, synthetic construct
GGIGDDTVN

SEQ ID NO: 44449 - protein, 9 aa, synthetic construct
GGIGDDVFS

SEQ ID NO: 44450 - protein, 9 aa, synthetic construct
GGIGDDVFY

SEQ ID NO: 44451 - protein, 9 aa, synthetic construct
GGIGDDVIA

SEQ ID NO: 44452 - protein, 9 aa, synthetic construct
GGIGDDVIN

SEQ ID NO: 44453 - protein, 9 aa, synthetic construct
GGIGDDVIY

SEQ ID NO: 44454 - protein, 9 aa, synthetic construct
GGIGDDVLG

SEQ ID NO: 44455 - protein, 9 aa, synthetic construct
GGIGDDVLK

SEQ ID NO: 44456 - protein, 9 aa, synthetic construct
GGIGDDVLL

SEQ ID NO: 44457 - protein, 9 aa, synthetic construct
GGIGDDVLT

SEQ ID NO: 44458 - protein, 9 aa, synthetic construct
GGIGDDVLV

SEQ ID NO: 44459 - protein, 9 aa, synthetic construct
GGIGDDVMI

SEQ ID NO: 44460 - protein, 9 aa, synthetic construct
GGIGDDVVN

SEQ ID NO: 44461 - protein, 9 aa, synthetic construct
GGIGDDWID

SEQ ID NO: 44462 - protein, 9 aa, synthetic construct
GGIGEDLLQ

SEQ ID NO: 44463 - protein, 9 aa, synthetic construct
GGIGDDWIE

SEQ ID NO: 44464 - protein, 9 aa, synthetic construct
GGIGDDWLN

SEQ ID NO: 44465 - protein, 9 aa, synthetic construct
GGIGDDWLV

SEQ ID NO: 44466 - protein, 9 aa, synthetic construct
GGIGDDYLA

SEQ ID NO: 44467 - protein, 9 aa, synthetic construct
GGIGDDYLH

SEQ ID NO: 44468 - protein, 9 aa, synthetic construct
GGIGDDYLL

SEQ ID NO: 44469 - protein, 9 aa, synthetic construct
GGIGDDYLT

SEQ ID NO: 44470 - protein, 9 aa, synthetic construct
GGIGEDALY

SEQ ID NO: 44471 - protein, 9 aa, synthetic construct
GGIGEDDYS

SEQ ID NO: 44472 - protein, 9 aa, synthetic construct
GGIGEDELI

SEQ ID NO: 44473 - protein, 9 aa, synthetic construct
GGIGEDELR

SEQ ID NO: 44474 - protein, 9 aa, synthetic construct
GGIGEDFLS

SEQ ID NO: 44475 - protein, 9 aa, synthetic construct
GGIGEDLLD

SEQ ID NO: 44476 - protein, 9 aa, synthetic construct
GGGGNDAVW

SEQ ID NO: 44477 - protein, 9 aa, synthetic construct
GGGGNDAVN

SEQ ID NO: 44478 - protein, 9 aa, synthetic construct
GGGGNDAMT

SEQ ID NO: 44479 - protein, 9 aa, synthetic construct
GGFGFDTLL

SEQ ID NO: 44480 - protein, 9 aa, synthetic construct
GGFGEDLLY

SEQ ID NO: 44481 - protein, 9 aa, synthetic construct
GGFGEDMLY

SEQ ID NO: 44482 - protein, 9 aa, synthetic construct
GGFGEDSIL

SEQ ID NO: 44483 - protein, 9 aa, synthetic construct
GGFGEDSLD

SEQ ID NO: 44484 - protein, 9 aa, synthetic construct
GGFGEDSLV

SEQ ID NO: 44485 - protein, 9 aa, synthetic construct
GGFGEDSLY

SEQ ID NO: 44486 - protein, 9 aa, synthetic construct
GGFGEDTII

SEQ ID NO: 44487 - protein, 9 aa, synthetic construct
GGFGEDTLD

SEQ ID NO: 44488 - protein, 9 aa, synthetic construct
GGFGEDTLF

SEQ ID NO: 44489 - protein, 9 aa, synthetic construct
GGFGEDTVV

SEQ ID NO: 44490 - protein, 9 aa, synthetic construct
GGFGEDVFL

SEQ ID NO: 44491 - protein, 9 aa, synthetic construct
GGFGEDVFV

SEQ ID NO: 44492 - protein, 9 aa, synthetic construct
GGFGEDVIF

SEQ ID NO: 44493 - protein, 9 aa, synthetic construct
GGFGEDVLS

SEQ ID NO: 44494 - protein, 9 aa, synthetic construct
GGFGFDIAN

SEQ ID NO: 44495 - protein, 9 aa, synthetic construct
GGFGFDLLN

SEQ ID NO: 44496 - protein, 9 aa, synthetic construct
GGFGFDLLS

SEQ ID NO: 44497 - protein, 9 aa, synthetic construct
GGFGFDQIF

SEQ ID NO: 44498 - protein, 9 aa, synthetic construct
GGFGFDRLF

SEQ ID NO: 44499 - protein, 9 aa, synthetic construct
GGFGFDRLI

SEQ ID NO: 44500 - protein, 9 aa, synthetic construct
GGFGFDRLK

SEQ ID NO: 44501 - protein, 9 aa, synthetic construct
GGFGFDRLS

SEQ ID NO: 44502 - protein, 9 aa, synthetic construct
GGFGFDRLV

SEQ ID NO: 44503 - protein, 9 aa, synthetic construct
GGFGFDRMT

SEQ ID NO: 44504 - protein, 9 aa, synthetic construct
GGFGFDRVG

SEQ ID NO: 44505 - protein, 9 aa, synthetic construct
GGFGFDSLN

SEQ ID NO: 44506 - protein, 9 aa, synthetic construct
GGFGFDTAE

SEQ ID NO: 44507 - protein, 9 aa, synthetic construct
GGFGFDTAF

SEQ ID NO: 44508 - protein, 9 aa, synthetic construct
GGFGFDTAH

SEQ ID NO: 44509 - protein, 9 aa, synthetic construct
GGFGEDLLS

SEQ ID NO: 44510 - protein, 9 aa, synthetic construct
GGFGEDLLR

SEQ ID NO: 44511 - protein, 9 aa, synthetic construct
GGFGEDLLQ

SEQ ID NO: 44512 - protein, 9 aa, synthetic construct
GGFGDDVYY

SEQ ID NO: 44513 - protein, 9 aa, synthetic construct
GGFGDDTVR

SEQ ID NO: 44514 - protein, 9 aa, synthetic construct
GGFGDDTVW

SEQ ID NO: 44515 - protein, 9 aa, synthetic construct
GGFGDDTYF

SEQ ID NO: 44516 - protein, 9 aa, synthetic construct
GGFGDDTYV

SEQ ID NO: 44517 - protein, 9 aa, synthetic construct
GGFGDDVAL

SEQ ID NO: 44518 - protein, 9 aa, synthetic construct
GGFGDDVFN

SEQ ID NO: 44519 - protein, 9 aa, synthetic construct
GGFGDDVFQ

SEQ ID NO: 44520 - protein, 9 aa, synthetic construct
GGFGDDVIE

SEQ ID NO: 44521 - protein, 9 aa, synthetic construct
GGFGDDVIG

SEQ ID NO: 44522 - protein, 9 aa, synthetic construct
GGFGDDVIR

SEQ ID NO: 44523 - protein, 9 aa, synthetic construct
GGFGDDVLE

SEQ ID NO: 44524 - protein, 9 aa, synthetic construct
GGFGDDVVR

SEQ ID NO: 44525 - protein, 9 aa, synthetic construct
GGFGDDVVS

SEQ ID NO: 44526 - protein, 9 aa, synthetic construct
GGFGDDWIA

SEQ ID NO: 44527 - protein, 9 aa, synthetic construct
GGFGEDLLN

SEQ ID NO: 44528 - protein, 9 aa, synthetic construct
GGFGDDWLD

SEQ ID NO: 44529 - protein, 9 aa, synthetic construct
GGFGDDYAE

SEQ ID NO: 44530 - protein, 9 aa, synthetic construct
GGFGDDYLD

SEQ ID NO: 44531 - protein, 9 aa, synthetic construct
GGFGDDYLE

SEQ ID NO: 44532 - protein, 9 aa, synthetic construct
GGFGEDALS

SEQ ID NO: 44533 - protein, 9 aa, synthetic construct
GGFGEDDLV

SEQ ID NO: 44534 - protein, 9 aa, synthetic construct
GGFGEDDMT

SEQ ID NO: 44535 - protein, 9 aa, synthetic construct
GGFGEDDVF

SEQ ID NO: 44536 - protein, 9 aa, synthetic construct
GGFGEDELI

SEQ ID NO: 44537 - protein, 9 aa, synthetic construct
GGFGEDELR

SEQ ID NO: 44538 - protein, 9 aa, synthetic construct
GGFGEDILQ

SEQ ID NO: 44539 - protein, 9 aa, synthetic construct
GGFGEDLIL

SEQ ID NO: 44540 - protein, 9 aa, synthetic construct
GGFGEDLLF

SEQ ID NO: 44541 - protein, 9 aa, synthetic construct
GGFGFDTFI

SEQ ID NO: 44542 - protein, 9 aa, synthetic construct
GGFGFDTYV

SEQ ID NO: 44543 - protein, 9 aa, synthetic construct
GGFGLDVAS

SEQ ID NO: 44544 - protein, 9 aa, synthetic construct
GGFGFDVLA

SEQ ID NO: 44545 - protein, 9 aa, synthetic construct
GGFGHDVVL

SEQ ID NO: 44546 - protein, 9 aa, synthetic construct
GGFGHDYLD

SEQ ID NO: 44547 - protein, 9 aa, synthetic construct
GGFGIDDLD

SEQ ID NO: 44548 - protein, 9 aa, synthetic construct
GGFGIDEIV

SEQ ID NO: 44549 - protein, 9 aa, synthetic construct
GGFGIDFLT

SEQ ID NO: 44550 - protein, 9 aa, synthetic construct
GGFGIDILD

SEQ ID NO: 44551 - protein, 9 aa, synthetic construct
GGFGIDILT

SEQ ID NO: 44552 - protein, 9 aa, synthetic construct
GGFGIDSLV

SEQ ID NO: 44553 - protein, 9 aa, synthetic construct
GGFGIDTAN

SEQ ID NO: 44554 - protein, 9 aa, synthetic construct
GGFGIDTLF

SEQ ID NO: 44555 - protein, 9 aa, synthetic construct
GGFGIDTLQ

SEQ ID NO: 44556 - protein, 9 aa, synthetic construct
GGFGIDTLT

SEQ ID NO: 44557 - protein, 9 aa, synthetic construct
GGFGIDTLY

SEQ ID NO: 44558 - protein, 9 aa, synthetic construct
GGFGIDTYF

SEQ ID NO: 44559 - protein, 9 aa, synthetic construct
GGFGIDYIY

SEQ ID NO: 44560 - protein, 9 aa, synthetic construct
GGFGIDYLD

SEQ ID NO: 44561 - protein, 9 aa, synthetic construct
GGFGKDILD

SEQ ID NO: 44562 - protein, 9 aa, synthetic construct
GGFGKDRIQ

SEQ ID NO: 44563 - protein, 9 aa, synthetic construct
GGFGKDSLV

SEQ ID NO: 44564 - protein, 9 aa, synthetic construct
GGFGKDTIN

SEQ ID NO: 44565 - protein, 9 aa, synthetic construct
GGFGKDTLL

SEQ ID NO: 44566 - protein, 9 aa, synthetic construct
GGFGKDVMS

SEQ ID NO: 44567 - protein, 9 aa, synthetic construct
GGFGLDLIA

SEQ ID NO: 44568 - protein, 9 aa, synthetic construct
GGFGLDRLW

SEQ ID NO: 44569 - protein, 9 aa, synthetic construct
GGFGLDSMI

SEQ ID NO: 44570 - protein, 9 aa, synthetic construct
GGFGLDTAH

SEQ ID NO: 44571 - protein, 9 aa, synthetic construct
GGFGLDTIN

SEQ ID NO: 44572 - protein, 9 aa, synthetic construct
GGFGLDTLL

SEQ ID NO: 44573 - protein, 9 aa, synthetic construct
GGFGLDTLM

SEQ ID NO: 44574 - protein, 9 aa, synthetic construct
GGFGHDVLN

SEQ ID NO: 44575 - protein, 9 aa, synthetic construct
GGFGHDVLM

SEQ ID NO: 44576 - protein, 9 aa, synthetic construct
GGFGHDVIY

SEQ ID NO: 44577 - protein, 9 aa, synthetic construct
GGFGGDTLS

SEQ ID NO: 44578 - protein, 9 aa, synthetic construct
GGFGFDVLF

SEQ ID NO: 44579 - protein, 9 aa, synthetic construct
GGFGFDVLT

SEQ ID NO: 44580 - protein, 9 aa, synthetic construct
GGFGGDAIE

SEQ ID NO: 44581 - protein, 9 aa, synthetic construct
GGFGGDAMR

SEQ ID NO: 44582 - protein, 9 aa, synthetic construct
GGFGGDCLF

SEQ ID NO: 44583 - protein, 9 aa, synthetic construct
GGFGGDGLY

SEQ ID NO: 44584 - protein, 9 aa, synthetic construct
GGFGGDRID

SEQ ID NO: 44585 - protein, 9 aa, synthetic construct
GGFGGDRLT

SEQ ID NO: 44586 - protein, 9 aa, synthetic construct
GGFGGDSLL

SEQ ID NO: 44587 - protein, 9 aa, synthetic construct
GGFGGDTIA

SEQ ID NO: 44588 - protein, 9 aa, synthetic construct
GGFGGDTIE

SEQ ID NO: 44589 - protein, 9 aa, synthetic construct
GGFGGDTII

SEQ ID NO: 44590 - protein, 9 aa, synthetic construct
GGFGGDTIT

SEQ ID NO: 44591 - protein, 9 aa, synthetic construct
GGFGGDVID

SEQ ID NO: 44592 - protein, 9 aa, synthetic construct
GGFGHDVII

SEQ ID NO: 44593 - protein, 9 aa, synthetic construct
GGFGGDVLH

SEQ ID NO: 44594 - protein, 9 aa, synthetic construct
GGFGHDAAF

SEQ ID NO: 44595 - protein, 9 aa, synthetic construct
GGFGHDMLA

SEQ ID NO: 44596 - protein, 9 aa, synthetic construct
GGFGHDQIY

SEQ ID NO: 44597 - protein, 9 aa, synthetic construct
GGFGHDRIE

SEQ ID NO: 44598 - protein, 9 aa, synthetic construct
GGFGHDRIS

SEQ ID NO: 44599 - protein, 9 aa, synthetic construct
GGFGHDRLL

SEQ ID NO: 44600 - protein, 9 aa, synthetic construct
GGFGHDRLM

SEQ ID NO: 44601 - protein, 9 aa, synthetic construct
GGFGHDRLY

SEQ ID NO: 44602 - protein, 9 aa, synthetic construct
GGFGHDTIY

SEQ ID NO: 44603 - protein, 9 aa, synthetic construct
GGFGHDTLN

SEQ ID NO: 44604 - protein, 9 aa, synthetic construct
GGFGHDTLR

SEQ ID NO: 44605 - protein, 9 aa, synthetic construct
GGFGHDTVT

SEQ ID NO: 44606 - protein, 9 aa, synthetic construct
GGFGDDTVK

SEQ ID NO: 44607 - protein, 9 aa, synthetic construct
GGFGDDTVH

SEQ ID NO: 44608 - protein, 9 aa, synthetic construct
GGFGDDTLQ

SEQ ID NO: 44609 - protein, 9 aa, synthetic construct
GGFGDDTLM

SEQ ID NO: 44610 - protein, 9 aa, synthetic construct
GGFGCDRVN

SEQ ID NO: 44611 - protein, 9 aa, synthetic construct
GGFGDDAIR

SEQ ID NO: 44612 - protein, 9 aa, synthetic construct
GGFGDDAIS

SEQ ID NO: 44613 - protein, 9 aa, synthetic construct
GGFGDDALD

SEQ ID NO: 44614 - protein, 9 aa, synthetic construct
GGFGDDALE

SEQ ID NO: 44615 - protein, 9 aa, synthetic construct
GGFGDDALK

SEQ ID NO: 44616 - protein, 9 aa, synthetic construct
GGFGDDAMH

SEQ ID NO: 44617 - protein, 9 aa, synthetic construct
GGFGDDAMN

SEQ ID NO: 44618 - protein, 9 aa, synthetic construct
GGFGDDAMT

SEQ ID NO: 44619 - protein, 9 aa, synthetic construct
GGFGDDAVL

SEQ ID NO: 44620 - protein, 9 aa, synthetic construct
GGFGDDAYK

SEQ ID NO: 44621 - protein, 9 aa, synthetic construct
GGFGDDDIK

SEQ ID NO: 44622 - protein, 9 aa, synthetic construct
GGFGDDDIT

SEQ ID NO: 44623 - protein, 9 aa, synthetic construct
GGFGDDDLR

SEQ ID NO: 44624 - protein, 9 aa, synthetic construct
GGFGDDEIG

SEQ ID NO: 44625 - protein, 9 aa, synthetic construct
GGFGDDELN

SEQ ID NO: 44626 - protein, 9 aa, synthetic construct
GGFGDDELS

SEQ ID NO: 44627 - protein, 9 aa, synthetic construct
GGFGDDELV

SEQ ID NO: 44628 - protein, 9 aa, synthetic construct
GGFGDDELW

SEQ ID NO: 44629 - protein, 9 aa, synthetic construct
GGFGDDEMS

SEQ ID NO: 44630 - protein, 9 aa, synthetic construct
GGFGDDFIN

SEQ ID NO: 44631 - protein, 9 aa, synthetic construct
GGFGDDFLI

SEQ ID NO: 44632 - protein, 9 aa, synthetic construct
GGFGDDFLL

SEQ ID NO: 44633 - protein, 9 aa, synthetic construct
GGFGDDFVD

SEQ ID NO: 44634 - protein, 9 aa, synthetic construct
GGFGDDFYF

SEQ ID NO: 44635 - protein, 9 aa, synthetic construct
GGFGDDGLT

SEQ ID NO: 44636 - protein, 9 aa, synthetic construct
GGFGDDGLY

SEQ ID NO: 44637 - protein, 9 aa, synthetic construct
GGFGDDGMG

SEQ ID NO: 44638 - protein, 9 aa, synthetic construct
GGFGDDHLD

SEQ ID NO: 44639 - protein, 9 aa, synthetic construct
GGFGADWLT

SEQ ID NO: 44640 - protein, 9 aa, synthetic construct
GGFGADWIE

SEQ ID NO: 44641 - protein, 9 aa, synthetic construct
GGFGADVVY

SEQ ID NO: 44642 - protein, 9 aa, synthetic construct
GGFGADTML

SEQ ID NO: 44643 - protein, 9 aa, synthetic construct
GGFGADSYI

SEQ ID NO: 44644 - protein, 9 aa, synthetic construct
GGFGADTFN

SEQ ID NO: 44645 - protein, 9 aa, synthetic construct
GGFGADTFY

SEQ ID NO: 44646 - protein, 9 aa, synthetic construct
GGFGADTIE

SEQ ID NO: 44647 - protein, 9 aa, synthetic construct
GGFGADTIF

SEQ ID NO: 44648 - protein, 9 aa, synthetic construct
GGFGADTIR

SEQ ID NO: 44649 - protein, 9 aa, synthetic construct
GGFGADTIS

SEQ ID NO: 44650 - protein, 9 aa, synthetic construct
GGFGADTIW

SEQ ID NO: 44651 - protein, 9 aa, synthetic construct
GGFGADTLK

SEQ ID NO: 44652 - protein, 9 aa, synthetic construct
GGFGADTLM

SEQ ID NO: 44653 - protein, 9 aa, synthetic construct
GGFGADTLV

SEQ ID NO: 44654 - protein, 9 aa, synthetic construct
GGFGADTME

SEQ ID NO: 44655 - protein, 9 aa, synthetic construct
GGFGADTMF

SEQ ID NO: 44656 - protein, 9 aa, synthetic construct
GGFGADTMR

SEQ ID NO: 44657 - protein, 9 aa, synthetic construct
GGFGADVVV

SEQ ID NO: 44658 - protein, 9 aa, synthetic construct
GGFGADTMV

SEQ ID NO: 44659 - protein, 9 aa, synthetic construct
GGFGADTVA

SEQ ID NO: 44660 - protein, 9 aa, synthetic construct
GGFGADTVF

SEQ ID NO: 44661 - protein, 9 aa, synthetic construct
GGFGADTYL

SEQ ID NO: 44662 - protein, 9 aa, synthetic construct
GGFGADVIH

SEQ ID NO: 44663 - protein, 9 aa, synthetic construct
GGFGADVIS

SEQ ID NO: 44664 - protein, 9 aa, synthetic construct
GGFGADVIY

SEQ ID NO: 44665 - protein, 9 aa, synthetic construct
GGFGADVLD

SEQ ID NO: 44666 - protein, 9 aa, synthetic construct
GGFGADVLH

SEQ ID NO: 44667 - protein, 9 aa, synthetic construct
GGFGADVLK

SEQ ID NO: 44668 - protein, 9 aa, synthetic construct
GGFGADVLN

SEQ ID NO: 44669 - protein, 9 aa, synthetic construct
GGFGADVLY

SEQ ID NO: 44670 - protein, 9 aa, synthetic construct
GGFGADVVM

SEQ ID NO: 44671 - protein, 9 aa, synthetic construct
GGFGDDHLI

SEQ ID NO: 44672 - protein, 9 aa, synthetic construct
GGFGDDHLN

SEQ ID NO: 44673 - protein, 9 aa, synthetic construct
GGFGDDIFV

SEQ ID NO: 44674 - protein, 9 aa, synthetic construct
GGFGDDSIT

SEQ ID NO: 44675 - protein, 9 aa, synthetic construct
GGFGDDQIW

SEQ ID NO: 44676 - protein, 9 aa, synthetic construct
GGFGDDQLD

SEQ ID NO: 44677 - protein, 9 aa, synthetic construct
GGFGDDQLE

SEQ ID NO: 44678 - protein, 9 aa, synthetic construct
GGFGDDQLF

SEQ ID NO: 44679 - protein, 9 aa, synthetic construct
GGFGDDRIE

SEQ ID NO: 44680 - protein, 9 aa, synthetic construct
GGFGDDRIW

SEQ ID NO: 44681 - protein, 9 aa, synthetic construct
GGFGDDRLS

SEQ ID NO: 44682 - protein, 9 aa, synthetic construct
GGFGDDRLT

SEQ ID NO: 44683 - protein, 9 aa, synthetic construct
GGFGDDRLW

SEQ ID NO: 44684 - protein, 9 aa, synthetic construct
GGFGDDRMH

SEQ ID NO: 44685 - protein, 9 aa, synthetic construct
GGFGDDSFF

SEQ ID NO: 44686 - protein, 9 aa, synthetic construct
GGFGDDSIA

SEQ ID NO: 44687 - protein, 9 aa, synthetic construct
GGFGDDSIE

SEQ ID NO: 44688 - protein, 9 aa, synthetic construct
GGFGDDSLD

SEQ ID NO: 44689 - protein, 9 aa, synthetic construct
GGFGDDQIT

SEQ ID NO: 44690 - protein, 9 aa, synthetic construct
GGFGDDSLG

SEQ ID NO: 44691 - protein, 9 aa, synthetic construct
GGFGDDSLR

SEQ ID NO: 44692 - protein, 9 aa, synthetic construct
GGFGDDSLS

SEQ ID NO: 44693 - protein, 9 aa, synthetic construct
GGFGDDSMD

SEQ ID NO: 44694 - protein, 9 aa, synthetic construct
GGFGDDSVK

SEQ ID NO: 44695 - protein, 9 aa, synthetic construct
GGFGDDSVS

SEQ ID NO: 44696 - protein, 9 aa, synthetic construct
GGFGDDSYN

SEQ ID NO: 44697 - protein, 9 aa, synthetic construct
GGFGDDTAS

SEQ ID NO: 44698 - protein, 9 aa, synthetic construct
GGFGDDTFH

SEQ ID NO: 44699 - protein, 9 aa, synthetic construct
GGFGDDTFY

SEQ ID NO: 44700 - protein, 9 aa, synthetic construct
GGFGDDTIN

SEQ ID NO: 44701 - protein, 9 aa, synthetic construct
GGFGDDTIQ

SEQ ID NO: 44702 - protein, 9 aa, synthetic construct
GGFGDDTLK

SEQ ID NO: 44703 - protein, 9 aa, synthetic construct
GGFGDDQIV

SEQ ID NO: 44704 - protein, 9 aa, synthetic construct
GGFGDDQIF

SEQ ID NO: 44705 - protein, 9 aa, synthetic construct
GGFGDDIID

SEQ ID NO: 44706 - protein, 9 aa, synthetic construct
GGFGDDLIW

SEQ ID NO: 44707 - protein, 9 aa, synthetic construct
GGFGDDIIN

SEQ ID NO: 44708 - protein, 9 aa, synthetic construct
GGFGDDILS

SEQ ID NO: 44709 - protein, 9 aa, synthetic construct
GGFGDDILY

SEQ ID NO: 44710 - protein, 9 aa, synthetic construct
GGFGDDIVR

SEQ ID NO: 44711 - protein, 9 aa, synthetic construct
GGFGDDIYV

SEQ ID NO: 44712 - protein, 9 aa, synthetic construct
GGFGDDIYY

SEQ ID NO: 44713 - protein, 9 aa, synthetic construct
GGFGDDKLF

SEQ ID NO: 44714 - protein, 9 aa, synthetic construct
GGFGDDLFD

SEQ ID NO: 44715 - protein, 9 aa, synthetic construct
GGFGDDLFV

SEQ ID NO: 44716 - protein, 9 aa, synthetic construct
GGFGDDLIA

SEQ ID NO: 44717 - protein, 9 aa, synthetic construct
GGFGDDLID

SEQ ID NO: 44718 - protein, 9 aa, synthetic construct
GGFGDDLIH

SEQ ID NO: 44719 - protein, 9 aa, synthetic construct
GGFGDDLII

SEQ ID NO: 44720 - protein, 9 aa, synthetic construct
GGFGDDLIY

SEQ ID NO: 44721 - protein, 9 aa, synthetic construct
GGFGDDPLI

SEQ ID NO: 44722 - protein, 9 aa, synthetic construct
GGFGDDLLC

SEQ ID NO: 44723 - protein, 9 aa, synthetic construct
GGFGDDLLF

SEQ ID NO: 44724 - protein, 9 aa, synthetic construct
GGFGDDLLG

SEQ ID NO: 44725 - protein, 9 aa, synthetic construct
GGFGDDLLR

SEQ ID NO: 44726 - protein, 9 aa, synthetic construct
GGFGDDLLV

SEQ ID NO: 44727 - protein, 9 aa, synthetic construct
GGFGDDLMI

SEQ ID NO: 44728 - protein, 9 aa, synthetic construct
GGFGDDLMT

SEQ ID NO: 44729 - protein, 9 aa, synthetic construct
GGFGDDLVR

SEQ ID NO: 44730 - protein, 9 aa, synthetic construct
GGFGDDLYR

SEQ ID NO: 44731 - protein, 9 aa, synthetic construct
GGFGDDMIM

SEQ ID NO: 44732 - protein, 9 aa, synthetic construct
GGFGDDMLA

SEQ ID NO: 44733 - protein, 9 aa, synthetic construct
GGFGDDNLD

SEQ ID NO: 44734 - protein, 9 aa, synthetic construct
GGFGDDNLY

SEQ ID NO: 44735 - protein, 9 aa, synthetic construct
GGFGLDTLN

SEQ ID NO: 44736 - protein, 9 aa, synthetic construct
GGFGLDVAV

SEQ ID NO: 44737 - protein, 9 aa, synthetic construct
GGFGVDILR

SEQ ID NO: 44738 - protein, 9 aa, synthetic construct
GGFGSDEVV

SEQ ID NO: 44739 - protein, 9 aa, synthetic construct
GGFGRDLLE

SEQ ID NO: 44740 - protein, 9 aa, synthetic construct
GGFGRDLLS

SEQ ID NO: 44741 - protein, 9 aa, synthetic construct
GGFGRDLVR

SEQ ID NO: 44742 - protein, 9 aa, synthetic construct
GGFGRDQIW

SEQ ID NO: 44743 - protein, 9 aa, synthetic construct
GGFGRDRIF

SEQ ID NO: 44744 - protein, 9 aa, synthetic construct
GGFGRDRLI

SEQ ID NO: 44745 - protein, 9 aa, synthetic construct
GGFGRDRLN

SEQ ID NO: 44746 - protein, 9 aa, synthetic construct
GGFGRDSIA

SEQ ID NO: 44747 - protein, 9 aa, synthetic construct
GGFGRDSIL

SEQ ID NO: 44748 - protein, 9 aa, synthetic construct
GGFGRDTAF

SEQ ID NO: 44749 - protein, 9 aa, synthetic construct
GGFGRDTFM

SEQ ID NO: 44750 - protein, 9 aa, synthetic construct
GGFGRDTID

SEQ ID NO: 44751 - protein, 9 aa, synthetic construct
GGFGRDTLA

SEQ ID NO: 44752 - protein, 9 aa, synthetic construct
GGFGRDTLD

SEQ ID NO: 44753 - protein, 9 aa, synthetic construct
GGFGRDTLL

SEQ ID NO: 44754 - protein, 9 aa, synthetic construct
GGFGRDTLQ

SEQ ID NO: 44755 - protein, 9 aa, synthetic construct
GGFGRDTLS

SEQ ID NO: 44756 - protein, 9 aa, synthetic construct
GGFGRDTLV

SEQ ID NO: 44757 - protein, 9 aa, synthetic construct
GGFGRDTLY

SEQ ID NO: 44758 - protein, 9 aa, synthetic construct
GGFGRDVFI

SEQ ID NO: 44759 - protein, 9 aa, synthetic construct
GGFGRDVFV

SEQ ID NO: 44760 - protein, 9 aa, synthetic construct
GGFGRDVLD

SEQ ID NO: 44761 - protein, 9 aa, synthetic construct
GGFGSDAIN

SEQ ID NO: 44762 - protein, 9 aa, synthetic construct
GGFGSDAIT

SEQ ID NO: 44763 - protein, 9 aa, synthetic construct
GGFGSDALF

SEQ ID NO: 44764 - protein, 9 aa, synthetic construct
GGFGSDAMW

SEQ ID NO: 44765 - protein, 9 aa, synthetic construct
GGFGSDAYI

SEQ ID NO: 44766 - protein, 9 aa, synthetic construct
GGFGSDDMS

SEQ ID NO: 44767 - protein, 9 aa, synthetic construct
GGFGSDELH

SEQ ID NO: 44768 - protein, 9 aa, synthetic construct
GGFGRDLLD

SEQ ID NO: 44769 - protein, 9 aa, synthetic construct
GGFGRDLIN

SEQ ID NO: 44770 - protein, 9 aa, synthetic construct
GGFGRDLIL

SEQ ID NO: 44771 - protein, 9 aa, synthetic construct
GGFGQDTLI

SEQ ID NO: 44772 - protein, 9 aa, synthetic construct
GGFGNDYIN

SEQ ID NO: 44773 - protein, 9 aa, synthetic construct
GGFGNDYLN

SEQ ID NO: 44774 - protein, 9 aa, synthetic construct
GGFGNDYLR

SEQ ID NO: 44775 - protein, 9 aa, synthetic construct
GGFGNDYLS

SEQ ID NO: 44776 - protein, 9 aa, synthetic construct
GGFGNDYLV

SEQ ID NO: 44777 - protein, 9 aa, synthetic construct
GGFGPDGLI

SEQ ID NO: 44778 - protein, 9 aa, synthetic construct
GGFGPDQLT

SEQ ID NO: 44779 - protein, 9 aa, synthetic construct
GGFGPDVLY

SEQ ID NO: 44780 - protein, 9 aa, synthetic construct
GGFGQDIIL

SEQ ID NO: 44781 - protein, 9 aa, synthetic construct
GGFGQDLID

SEQ ID NO: 44782 - protein, 9 aa, synthetic construct
GGFGQDLLT

SEQ ID NO: 44783 - protein, 9 aa, synthetic construct
GGFGQDLLY

SEQ ID NO: 44784 - protein, 9 aa, synthetic construct
GGFGQDTLF

SEQ ID NO: 44785 - protein, 9 aa, synthetic construct
GGFGQDTLS

SEQ ID NO: 44786 - protein, 9 aa, synthetic construct
GGFGRDLAR

SEQ ID NO: 44787 - protein, 9 aa, synthetic construct
GGFGQDTLV

SEQ ID NO: 44788 - protein, 9 aa, synthetic construct
GGFGQDTVI

SEQ ID NO: 44789 - protein, 9 aa, synthetic construct
GGFGQDTVS

SEQ ID NO: 44790 - protein, 9 aa, synthetic construct
GGFGQDVLE

SEQ ID NO: 44791 - protein, 9 aa, synthetic construct
GGFGQDWVV

SEQ ID NO: 44792 - protein, 9 aa, synthetic construct
GGFGQDYLF

SEQ ID NO: 44793 - protein, 9 aa, synthetic construct
GGFGRDAIS

SEQ ID NO: 44794 - protein, 9 aa, synthetic construct
GGFGRDALN

SEQ ID NO: 44795 - protein, 9 aa, synthetic construct
GGFGRDFYY

SEQ ID NO: 44796 - protein, 9 aa, synthetic construct
GGFGRDILR

SEQ ID NO: 44797 - protein, 9 aa, synthetic construct
GGFGRDILV

SEQ ID NO: 44798 - protein, 9 aa, synthetic construct
GGFGRDIMT

SEQ ID NO: 44799 - protein, 9 aa, synthetic construct
GGFGRDKLW

SEQ ID NO: 44800 - protein, 9 aa, synthetic construct
GGFGSDELI

SEQ ID NO: 44801 - protein, 9 aa, synthetic construct
GGFGSDFLF

SEQ ID NO: 44802 - protein, 9 aa, synthetic construct
GGFGLDYIQ

SEQ ID NO: 44803 - protein, 9 aa, synthetic construct
GGFGSDHMQ

SEQ ID NO: 44804 - protein, 9 aa, synthetic construct
GGFGSDVFA

SEQ ID NO: 44805 - protein, 9 aa, synthetic construct
GGFGSDVIL

SEQ ID NO: 44806 - protein, 9 aa, synthetic construct
GGFGSDVLA

SEQ ID NO: 44807 - protein, 9 aa, synthetic construct
GGFGSDVLD

SEQ ID NO: 44808 - protein, 9 aa, synthetic construct
GGFGSDVLE

SEQ ID NO: 44809 - protein, 9 aa, synthetic construct
GGFGSDVLF

SEQ ID NO: 44810 - protein, 9 aa, synthetic construct
GGFGSDVLI

SEQ ID NO: 44811 - protein, 9 aa, synthetic construct
GGFGSDVLR

SEQ ID NO: 44812 - protein, 9 aa, synthetic construct
GGFGSDVLT

SEQ ID NO: 44813 - protein, 9 aa, synthetic construct
GGFGSDYLS

SEQ ID NO: 44814 - protein, 9 aa, synthetic construct
GGFGSDYMV

SEQ ID NO: 44815 - protein, 9 aa, synthetic construct
GGFGTDFLI

SEQ ID NO: 44816 - protein, 9 aa, synthetic construct
GGFGTDILT

SEQ ID NO: 44817 - protein, 9 aa, synthetic construct
GGFGTDKLI

SEQ ID NO: 44818 - protein, 9 aa, synthetic construct
GGFGTDLLI

SEQ ID NO: 44819 - protein, 9 aa, synthetic construct
GGFGTDNLS

SEQ ID NO: 44820 - protein, 9 aa, synthetic construct
GGFGTDRVD

SEQ ID NO: 44821 - protein, 9 aa, synthetic construct
GGFGTDRVE

SEQ ID NO: 44822 - protein, 9 aa, synthetic construct
GGFGTDSLA

SEQ ID NO: 44823 - protein, 9 aa, synthetic construct
GGFGTDTFV

SEQ ID NO: 44824 - protein, 9 aa, synthetic construct
GGFGTDTIA

SEQ ID NO: 44825 - protein, 9 aa, synthetic construct
GGFGTDTLK

SEQ ID NO: 44826 - protein, 9 aa, synthetic construct
GGFGTDTLL

SEQ ID NO: 44827 - protein, 9 aa, synthetic construct
GGFGTDTLN

SEQ ID NO: 44828 - protein, 9 aa, synthetic construct
GGFGTDTVT

SEQ ID NO: 44829 - protein, 9 aa, synthetic construct
GGFGTDYMA

SEQ ID NO: 44830 - protein, 9 aa, synthetic construct
GGFGVDHIF

SEQ ID NO: 44831 - protein, 9 aa, synthetic construct
GGFGVDHVH

SEQ ID NO: 44832 - protein, 9 aa, synthetic construct
GGFGVDIIA

SEQ ID NO: 44833 - protein, 9 aa, synthetic construct
GGFGSDTYR

SEQ ID NO: 44834 - protein, 9 aa, synthetic construct
GGFGSDTLS

SEQ ID NO: 44835 - protein, 9 aa, synthetic construct
GGFGSDTLN

SEQ ID NO: 44836 - protein, 9 aa, synthetic construct
GGFGSDLLY

SEQ ID NO: 44837 - protein, 9 aa, synthetic construct
GGFGSDIIN

SEQ ID NO: 44838 - protein, 9 aa, synthetic construct
GGFGSDIIR

SEQ ID NO: 44839 - protein, 9 aa, synthetic construct
GGFGSDILI

SEQ ID NO: 44840 - protein, 9 aa, synthetic construct
GGFGSDILS

SEQ ID NO: 44841 - protein, 9 aa, synthetic construct
GGFGSDILT

SEQ ID NO: 44842 - protein, 9 aa, synthetic construct
GGFGSDIYY

SEQ ID NO: 44843 - protein, 9 aa, synthetic construct
GGFGSDKIT

SEQ ID NO: 44844 - protein, 9 aa, synthetic construct
GGFGSDKLI

SEQ ID NO: 44845 - protein, 9 aa, synthetic construct
GGFGSDKLS

SEQ ID NO: 44846 - protein, 9 aa, synthetic construct
GGFGSDLFH

SEQ ID NO: 44847 - protein, 9 aa, synthetic construct
GGFGSDLFV

SEQ ID NO: 44848 - protein, 9 aa, synthetic construct
GGFGSDLLN

SEQ ID NO: 44849 - protein, 9 aa, synthetic construct
GGFGSDLLT

SEQ ID NO: 44850 - protein, 9 aa, synthetic construct
GGFGSDQIV

SEQ ID NO: 44851 - protein, 9 aa, synthetic construct
GGFGSDTLK

SEQ ID NO: 44852 - protein, 9 aa, synthetic construct
GGFGSDQVL

SEQ ID NO: 44853 - protein, 9 aa, synthetic construct
GGFGSDRIH

SEQ ID NO: 44854 - protein, 9 aa, synthetic construct
GGFGSDRLF

SEQ ID NO: 44855 - protein, 9 aa, synthetic construct
GGFGSDRLT

SEQ ID NO: 44856 - protein, 9 aa, synthetic construct
GGFGSDRLV

SEQ ID NO: 44857 - protein, 9 aa, synthetic construct
GGFGSDRMV

SEQ ID NO: 44858 - protein, 9 aa, synthetic construct
GGFGSDSLD

SEQ ID NO: 44859 - protein, 9 aa, synthetic construct
GGFGSDSLE

SEQ ID NO: 44860 - protein, 9 aa, synthetic construct
GGFGSDSLI

SEQ ID NO: 44861 - protein, 9 aa, synthetic construct
GGFGSDSLV

SEQ ID NO: 44862 - protein, 9 aa, synthetic construct
GGFGSDTAD

SEQ ID NO: 44863 - protein, 9 aa, synthetic construct
GGFGSDTLE

SEQ ID NO: 44864 - protein, 9 aa, synthetic construct
GGFGSDTLG

SEQ ID NO: 44865 - protein, 9 aa, synthetic construct
GGFGNDWLQ

SEQ ID NO: 44866 - protein, 9 aa, synthetic construct
GGFGNDWIG

SEQ ID NO: 44867 - protein, 9 aa, synthetic construct
GGFGNDVYL

SEQ ID NO: 44868 - protein, 9 aa, synthetic construct
GGFGNDVVV

SEQ ID NO: 44869 - protein, 9 aa, synthetic construct
GGFGNDGLS

SEQ ID NO: 44870 - protein, 9 aa, synthetic construct
GGFGNDHLE

SEQ ID NO: 44871 - protein, 9 aa, synthetic construct
GGFGNDHLF

SEQ ID NO: 44872 - protein, 9 aa, synthetic construct
GGFGNDHLV

SEQ ID NO: 44873 - protein, 9 aa, synthetic construct
GGFGNDHMW

SEQ ID NO: 44874 - protein, 9 aa, synthetic construct
GGFGNDIAN

SEQ ID NO: 44875 - protein, 9 aa, synthetic construct
GGFGNDIII

SEQ ID NO: 44876 - protein, 9 aa, synthetic construct
GGFGNDIIL

SEQ ID NO: 44877 - protein, 9 aa, synthetic construct
GGFGNDILA

SEQ ID NO: 44878 - protein, 9 aa, synthetic construct
GGFGNDILD

SEQ ID NO: 44879 - protein, 9 aa, synthetic construct
GGFGNDILH

SEQ ID NO: 44880 - protein, 9 aa, synthetic construct
GGFGNDILQ

SEQ ID NO: 44881 - protein, 9 aa, synthetic construct
GGFGNDILS

SEQ ID NO: 44882 - protein, 9 aa, synthetic construct
GGFGNDILV

SEQ ID NO: 44883 - protein, 9 aa, synthetic construct
GGFGNDIMD

SEQ ID NO: 44884 - protein, 9 aa, synthetic construct
GGFGNDIMV

SEQ ID NO: 44885 - protein, 9 aa, synthetic construct
GGFGNDIVL

SEQ ID NO: 44886 - protein, 9 aa, synthetic construct
GGFGNDIYF

SEQ ID NO: 44887 - protein, 9 aa, synthetic construct
GGFGNDIYR

SEQ ID NO: 44888 - protein, 9 aa, synthetic construct
GGFGNDKIG

SEQ ID NO: 44889 - protein, 9 aa, synthetic construct
GGFGNDKLV

SEQ ID NO: 44890 - protein, 9 aa, synthetic construct
GGFGNDKVD

SEQ ID NO: 44891 - protein, 9 aa, synthetic construct
GGFGNDLIE

SEQ ID NO: 44892 - protein, 9 aa, synthetic construct
GGFGNDLIV

SEQ ID NO: 44893 - protein, 9 aa, synthetic construct
GGFGNDLIW

SEQ ID NO: 44894 - protein, 9 aa, synthetic construct
GGFGNDLLD

SEQ ID NO: 44895 - protein, 9 aa, synthetic construct
GGFGNDLLE

SEQ ID NO: 44896 - protein, 9 aa, synthetic construct
GGFGNDLLH

SEQ ID NO: 44897 - protein, 9 aa, synthetic construct
GGFGNDLLQ

SEQ ID NO: 44898 - protein, 9 aa, synthetic construct
GGFGNDGLN

SEQ ID NO: 44899 - protein, 9 aa, synthetic construct
GGFGNDFVD

SEQ ID NO: 44900 - protein, 9 aa, synthetic construct
GGFGNDFLY

SEQ ID NO: 44901 - protein, 9 aa, synthetic construct
GGFGNDDIF

SEQ ID NO: 44902 - protein, 9 aa, synthetic construct
GGFGMDLLD

SEQ ID NO: 44903 - protein, 9 aa, synthetic construct
GGFGMDLVE

SEQ ID NO: 44904 - protein, 9 aa, synthetic construct
GGFGMDTLV

SEQ ID NO: 44905 - protein, 9 aa, synthetic construct
GGFGMDTVE

SEQ ID NO: 44906 - protein, 9 aa, synthetic construct
GGFGNDALA

SEQ ID NO: 44907 - protein, 9 aa, synthetic construct
GGFGNDALD

SEQ ID NO: 44908 - protein, 9 aa, synthetic construct
GGFGNDALE

SEQ ID NO: 44909 - protein, 9 aa, synthetic construct
GGFGNDALQ

SEQ ID NO: 44910 - protein, 9 aa, synthetic construct
GGFGNDALV

SEQ ID NO: 44911 - protein, 9 aa, synthetic construct
GGFGNDALY

SEQ ID NO: 44912 - protein, 9 aa, synthetic construct
GGFGNDAVA

SEQ ID NO: 44913 - protein, 9 aa, synthetic construct
GGFGNDAVL

SEQ ID NO: 44914 - protein, 9 aa, synthetic construct
GGFGNDAVT

SEQ ID NO: 44915 - protein, 9 aa, synthetic construct
GGFGNDDIY

SEQ ID NO: 44916 - protein, 9 aa, synthetic construct
GGFGNDFLQ

SEQ ID NO: 44917 - protein, 9 aa, synthetic construct
GGFGNDDLD

SEQ ID NO: 44918 - protein, 9 aa, synthetic construct
GGFGNDDLE

SEQ ID NO: 44919 - protein, 9 aa, synthetic construct
GGFGNDDLL

SEQ ID NO: 44920 - protein, 9 aa, synthetic construct
GGFGNDDLN

SEQ ID NO: 44921 - protein, 9 aa, synthetic construct
GGFGNDDVR

SEQ ID NO: 44922 - protein, 9 aa, synthetic construct
GGFGNDEIT

SEQ ID NO: 44923 - protein, 9 aa, synthetic construct
GGFGNDELD

SEQ ID NO: 44924 - protein, 9 aa, synthetic construct
GGFGNDELH

SEQ ID NO: 44925 - protein, 9 aa, synthetic construct
GGFGNDELT

SEQ ID NO: 44926 - protein, 9 aa, synthetic construct
GGFGNDEMF

SEQ ID NO: 44927 - protein, 9 aa, synthetic construct
GGFGNDEVD

SEQ ID NO: 44928 - protein, 9 aa, synthetic construct
GGFGNDEVN

SEQ ID NO: 44929 - protein, 9 aa, synthetic construct
GGFGNDFFR

SEQ ID NO: 44930 - protein, 9 aa, synthetic construct
GGFGNDLMI

SEQ ID NO: 44931 - protein, 9 aa, synthetic construct
GGFGNDLML

SEQ ID NO: 44932 - protein, 9 aa, synthetic construct
GGFGNDLMN

SEQ ID NO: 44933 - protein, 9 aa, synthetic construct
GGFGNDTVD

SEQ ID NO: 44934 - protein, 9 aa, synthetic construct
GGFGNDSVY

SEQ ID NO: 44935 - protein, 9 aa, synthetic construct
GGFGNDSYM

SEQ ID NO: 44936 - protein, 9 aa, synthetic construct
GGFGNDTAW

SEQ ID NO: 44937 - protein, 9 aa, synthetic construct
GGFGNDTFF

SEQ ID NO: 44938 - protein, 9 aa, synthetic construct
GGFGNDTFR

SEQ ID NO: 44939 - protein, 9 aa, synthetic construct
GGFGNDTFV

SEQ ID NO: 44940 - protein, 9 aa, synthetic construct
GGFGNDTIR

SEQ ID NO: 44941 - protein, 9 aa, synthetic construct
GGFGNDTIW

SEQ ID NO: 44942 - protein, 9 aa, synthetic construct
GGFGNDTLM

SEQ ID NO: 44943 - protein, 9 aa, synthetic construct
GGFGNDTLW

SEQ ID NO: 44944 - protein, 9 aa, synthetic construct
GGFGNDTMF

SEQ ID NO: 44945 - protein, 9 aa, synthetic construct
GGFGNDTML

SEQ ID NO: 44946 - protein, 9 aa, synthetic construct
GGFGNDTMT

SEQ ID NO: 44947 - protein, 9 aa, synthetic construct
GGFGNDTVI

SEQ ID NO: 44948 - protein, 9 aa, synthetic construct
GGFGNDSME

SEQ ID NO: 44949 - protein, 9 aa, synthetic construct
GGFGNDTYT

SEQ ID NO: 44950 - protein, 9 aa, synthetic construct
GGFGNDVFK

SEQ ID NO: 44951 - protein, 9 aa, synthetic construct
GGFGNDVFQ

SEQ ID NO: 44952 - protein, 9 aa, synthetic construct
GGFGNDVID

SEQ ID NO: 44953 - protein, 9 aa, synthetic construct
GGFGNDVIH

SEQ ID NO: 44954 - protein, 9 aa, synthetic construct
GGFGNDVIL

SEQ ID NO: 44955 - protein, 9 aa, synthetic construct
GGFGNDVIR

SEQ ID NO: 44956 - protein, 9 aa, synthetic construct
GGFGNDVIY

SEQ ID NO: 44957 - protein, 9 aa, synthetic construct
GGFGNDVLG

SEQ ID NO: 44958 - protein, 9 aa, synthetic construct
GGFGNDVLK

SEQ ID NO: 44959 - protein, 9 aa, synthetic construct
GGFGNDVLY

SEQ ID NO: 44960 - protein, 9 aa, synthetic construct
GGFGNDVMY

SEQ ID NO: 44961 - protein, 9 aa, synthetic construct
GGFGNDVVN

SEQ ID NO: 44962 - protein, 9 aa, synthetic construct
GGFGNDSVE

SEQ ID NO: 44963 - protein, 9 aa, synthetic construct
GGFGNDSLL

SEQ ID NO: 44964 - protein, 9 aa, synthetic construct
GGFGNDLMY

SEQ ID NO: 44965 - protein, 9 aa, synthetic construct
GGFGNDRIE

SEQ ID NO: 44966 - protein, 9 aa, synthetic construct
GGFGNDLVR

SEQ ID NO: 44967 - protein, 9 aa, synthetic construct
GGFGNDMIH

SEQ ID NO: 44968 - protein, 9 aa, synthetic construct
GGFGNDMIL

SEQ ID NO: 44969 - protein, 9 aa, synthetic construct
GGFGNDMLM

SEQ ID NO: 44970 - protein, 9 aa, synthetic construct
GGFGNDMLY

SEQ ID NO: 44971 - protein, 9 aa, synthetic construct
GGFGNDNLD

SEQ ID NO: 44972 - protein, 9 aa, synthetic construct
GGFGNDNLG

SEQ ID NO: 44973 - protein, 9 aa, synthetic construct
GGFGNDPLW

SEQ ID NO: 44974 - protein, 9 aa, synthetic construct
GGFGNDQLE

SEQ ID NO: 44975 - protein, 9 aa, synthetic construct
GGFGNDQLF

SEQ ID NO: 44976 - protein, 9 aa, synthetic construct
GGFGNDQLK

SEQ ID NO: 44977 - protein, 9 aa, synthetic construct
GGFGNDQMF

SEQ ID NO: 44978 - protein, 9 aa, synthetic construct
GGFGNDRAG

SEQ ID NO: 44979 - protein, 9 aa, synthetic construct
GGFGNDRIF

SEQ ID NO: 44980 - protein, 9 aa, synthetic construct
GGFGNDSLA

SEQ ID NO: 44981 - protein, 9 aa, synthetic construct
GGFGNDRIL

SEQ ID NO: 44982 - protein, 9 aa, synthetic construct
GGFGNDRIN

SEQ ID NO: 44983 - protein, 9 aa, synthetic construct
GGFGNDRLA

SEQ ID NO: 44984 - protein, 9 aa, synthetic construct
GGFGNDRLM

SEQ ID NO: 44985 - protein, 9 aa, synthetic construct
GGFGNDRLQ

SEQ ID NO: 44986 - protein, 9 aa, synthetic construct
GGFGNDRMY

SEQ ID NO: 44987 - protein, 9 aa, synthetic construct
GGFGNDRVN

SEQ ID NO: 44988 - protein, 9 aa, synthetic construct
GGFGNDRYV

SEQ ID NO: 44989 - protein, 9 aa, synthetic construct
GGFGNDSFA

SEQ ID NO: 44990 - protein, 9 aa, synthetic construct
GGFGNDSFS

SEQ ID NO: 44991 - protein, 9 aa, synthetic construct
GGFGNDSIF

SEQ ID NO: 44992 - protein, 9 aa, synthetic construct
GGFGNDSII

SEQ ID NO: 44993 - protein, 9 aa, synthetic construct
GGFGNDSIV

SEQ ID NO: 44994 - protein, 9 aa, synthetic construct
GGFGADSVT

SEQ ID NO: 44995 - protein, 9 aa, synthetic construct
GGFGADSVF

SEQ ID NO: 44996 - protein, 9 aa, synthetic construct
GGFGADSMT

SEQ ID NO: 44997 - protein, 9 aa, synthetic construct
GGEGSDLMV

SEQ ID NO: 44998 - protein, 9 aa, synthetic construct
GGEGSDIFF

SEQ ID NO: 44999 - protein, 9 aa, synthetic construct
GGEGSDIFL

SEQ ID NO: 45000 - protein, 9 aa, synthetic construct
GGEGSDIFR

SEQ ID NO: 45001 - protein, 9 aa, synthetic construct
GGEGSDIFS

SEQ ID NO: 45002 - protein, 9 aa, synthetic construct
GGEGSDIIE

SEQ ID NO: 45003 - protein, 9 aa, synthetic construct
GGEGSDIII

SEQ ID NO: 45004 - protein, 9 aa, synthetic construct
GGEGSDIIL

SEQ ID NO: 45005 - protein, 9 aa, synthetic construct
GGEGSDIIN

SEQ ID NO: 45006 - protein, 9 aa, synthetic construct
GGEGSDILC

SEQ ID NO: 45007 - protein, 9 aa, synthetic construct
GGEGSDILD

SEQ ID NO: 45008 - protein, 9 aa, synthetic construct
GGEGSDILF

SEQ ID NO: 45009 - protein, 9 aa, synthetic construct
GGEGSDILL

SEQ ID NO: 45010 - protein, 9 aa, synthetic construct
GGEGSDILT

SEQ ID NO: 45011 - protein, 9 aa, synthetic construct
GGEGSDILY

SEQ ID NO: 45012 - protein, 9 aa, synthetic construct
GGEGSDIVA

SEQ ID NO: 45013 - protein, 9 aa, synthetic construct
GGEGSDIYL

SEQ ID NO: 45014 - protein, 9 aa, synthetic construct
GGEGSDIYM

SEQ ID NO: 45015 - protein, 9 aa, synthetic construct
GGEGSDIYR

SEQ ID NO: 45016 - protein, 9 aa, synthetic construct
GGEGSDKFF

SEQ ID NO: 45017 - protein, 9 aa, synthetic construct
GGEGSDKLV

SEQ ID NO: 45018 - protein, 9 aa, synthetic construct
GGEGSDLFA

SEQ ID NO: 45019 - protein, 9 aa, synthetic construct
GGEGSDLFK

SEQ ID NO: 45020 - protein, 9 aa, synthetic construct
GGEGSDLFQ

SEQ ID NO: 45021 - protein, 9 aa, synthetic construct
GGEGSDLFV

SEQ ID NO: 45022 - protein, 9 aa, synthetic construct
GGEGSDLIL

SEQ ID NO: 45023 - protein, 9 aa, synthetic construct
GGEGSDLIT

SEQ ID NO: 45024 - protein, 9 aa, synthetic construct
GGEGSDLIV

SEQ ID NO: 45025 - protein, 9 aa, synthetic construct
GGEGSDLIY

SEQ ID NO: 45026 - protein, 9 aa, synthetic construct
GGEGSDLLF

SEQ ID NO: 45027 - protein, 9 aa, synthetic construct
GGEGSDIAS

SEQ ID NO: 45028 - protein, 9 aa, synthetic construct
GGEGSDIAQ

SEQ ID NO: 45029 - protein, 9 aa, synthetic construct
GGEGSDHMY

SEQ ID NO: 45030 - protein, 9 aa, synthetic construct
GGEGSDFID

SEQ ID NO: 45031 - protein, 9 aa, synthetic construct
GGEGSDALK

SEQ ID NO: 45032 - protein, 9 aa, synthetic construct
GGEGSDALN

SEQ ID NO: 45033 - protein, 9 aa, synthetic construct
GGEGSDAYA

SEQ ID NO: 45034 - protein, 9 aa, synthetic construct
GGEGSDAYL

SEQ ID NO: 45035 - protein, 9 aa, synthetic construct
GGEGSDDIL

SEQ ID NO: 45036 - protein, 9 aa, synthetic construct
GGEGSDDLK

SEQ ID NO: 45037 - protein, 9 aa, synthetic construct
GGEGSDDLR

SEQ ID NO: 45038 - protein, 9 aa, synthetic construct
GGEGSDDLY

SEQ ID NO: 45039 - protein, 9 aa, synthetic construct
GGEGSDEIH

SEQ ID NO: 45040 - protein, 9 aa, synthetic construct
GGEGSDELF

SEQ ID NO: 45041 - protein, 9 aa, synthetic construct
GGEGSDELI

SEQ ID NO: 45042 - protein, 9 aa, synthetic construct
GGEGSDELL

SEQ ID NO: 45043 - protein, 9 aa, synthetic construct
GGEGSDELR

SEQ ID NO: 45044 - protein, 9 aa, synthetic construct
GGEGSDFIQ

SEQ ID NO: 45045 - protein, 9 aa, synthetic construct
GGEGSDHMR

SEQ ID NO: 45046 - protein, 9 aa, synthetic construct
GGEGSDFLL

SEQ ID NO: 45047 - protein, 9 aa, synthetic construct
GGEGSDFLQ

SEQ ID NO: 45048 - protein, 9 aa, synthetic construct
GGEGSDFLV

SEQ ID NO: 45049 - protein, 9 aa, synthetic construct
GGEGSDFLY

SEQ ID NO: 45050 - protein, 9 aa, synthetic construct
GGEGSDFYI

SEQ ID NO: 45051 - protein, 9 aa, synthetic construct
GGEGSDGLH

SEQ ID NO: 45052 - protein, 9 aa, synthetic construct
GGEGSDGLR

SEQ ID NO: 45053 - protein, 9 aa, synthetic construct
GGEGSDHFV

SEQ ID NO: 45054 - protein, 9 aa, synthetic construct
GGEGSDHIH

SEQ ID NO: 45055 - protein, 9 aa, synthetic construct
GGEGSDHLI

SEQ ID NO: 45056 - protein, 9 aa, synthetic construct
GGEGSDHLS

SEQ ID NO: 45057 - protein, 9 aa, synthetic construct
GGEGSDHLY

SEQ ID NO: 45058 - protein, 9 aa, synthetic construct
GGEGSDHMD

SEQ ID NO: 45059 - protein, 9 aa, synthetic construct
GGEGSDLLM

SEQ ID NO: 45060 - protein, 9 aa, synthetic construct
GGEGSDLVE

SEQ ID NO: 45061 - protein, 9 aa, synthetic construct
GGFGADSME

SEQ ID NO: 45062 - protein, 9 aa, synthetic construct
GGEGSDMLL

SEQ ID NO: 45063 - protein, 9 aa, synthetic construct
GGEGSDSVE

SEQ ID NO: 45064 - protein, 9 aa, synthetic construct
GGEGSDTAL

SEQ ID NO: 45065 - protein, 9 aa, synthetic construct
GGEGSDTAR

SEQ ID NO: 45066 - protein, 9 aa, synthetic construct
GGEGSDTAV

SEQ ID NO: 45067 - protein, 9 aa, synthetic construct
GGEGSDTFA

SEQ ID NO: 45068 - protein, 9 aa, synthetic construct
GGEGSDTFR

SEQ ID NO: 45069 - protein, 9 aa, synthetic construct
GGEGSDTFT

SEQ ID NO: 45070 - protein, 9 aa, synthetic construct
GGEGSDTIM

SEQ ID NO: 45071 - protein, 9 aa, synthetic construct
GGEGSDTIR

SEQ ID NO: 45072 - protein, 9 aa, synthetic construct
GGEGSDTIT

SEQ ID NO: 45073 - protein, 9 aa, synthetic construct
GGEGSDTLF

SEQ ID NO: 45074 - protein, 9 aa, synthetic construct
GGEGSDTLG

SEQ ID NO: 45075 - protein, 9 aa, synthetic construct
GGEGSDTLH

SEQ ID NO: 45076 - protein, 9 aa, synthetic construct
GGEGSDTMG

SEQ ID NO: 45077 - protein, 9 aa, synthetic construct
GGEGSDTMR

SEQ ID NO: 45078 - protein, 9 aa, synthetic construct
GGEGSDTVI

SEQ ID NO: 45079 - protein, 9 aa, synthetic construct
GGEGSDTVR

SEQ ID NO: 45080 - protein, 9 aa, synthetic construct
GGEGSDTVV

SEQ ID NO: 45081 - protein, 9 aa, synthetic construct
GGEGSDTVY

SEQ ID NO: 45082 - protein, 9 aa, synthetic construct
GGEGSDTYH

SEQ ID NO: 45083 - protein, 9 aa, synthetic construct
GGEGSDTYK

SEQ ID NO: 45084 - protein, 9 aa, synthetic construct
GGEGSDVFL

SEQ ID NO: 45085 - protein, 9 aa, synthetic construct
GGEGSDVFT

SEQ ID NO: 45086 - protein, 9 aa, synthetic construct
GGEGSDVFY

SEQ ID NO: 45087 - protein, 9 aa, synthetic construct
GGEGSDVIF

SEQ ID NO: 45088 - protein, 9 aa, synthetic construct
GGEGSDVIK

SEQ ID NO: 45089 - protein, 9 aa, synthetic construct
GGEGSDVIY

SEQ ID NO: 45090 - protein, 9 aa, synthetic construct
GGEGSDVLK

SEQ ID NO: 45091 - protein, 9 aa, synthetic construct
GGEGSDVLY

SEQ ID NO: 45092 - protein, 9 aa, synthetic construct
GGEGSDSVD

SEQ ID NO: 45093 - protein, 9 aa, synthetic construct
GGEGSDSLS

SEQ ID NO: 45094 - protein, 9 aa, synthetic construct
GGEGSDSLR

SEQ ID NO: 45095 - protein, 9 aa, synthetic construct
GGEGSDRAM

SEQ ID NO: 45096 - protein, 9 aa, synthetic construct
GGEGSDMLV

SEQ ID NO: 45097 - protein, 9 aa, synthetic construct
GGEGSDMLW

SEQ ID NO: 45098 - protein, 9 aa, synthetic construct
GGEGSDMLY

SEQ ID NO: 45099 - protein, 9 aa, synthetic construct
GGEGSDNFY

SEQ ID NO: 45100 - protein, 9 aa, synthetic construct
GGEGSDNLI

SEQ ID NO: 45101 - protein, 9 aa, synthetic construct
GGEGSDNLY

SEQ ID NO: 45102 - protein, 9 aa, synthetic construct
GGEGSDNMD

SEQ ID NO: 45103 - protein, 9 aa, synthetic construct
GGEGSDQIW

SEQ ID NO: 45104 - protein, 9 aa, synthetic construct
GGEGSDQLA

SEQ ID NO: 45105 - protein, 9 aa, synthetic construct
GGEGSDQLH

SEQ ID NO: 45106 - protein, 9 aa, synthetic construct
GGEGSDQLL

SEQ ID NO: 45107 - protein, 9 aa, synthetic construct
GGEGSDQLT

SEQ ID NO: 45108 - protein, 9 aa, synthetic construct
GGEGSDQLV

SEQ ID NO: 45109 - protein, 9 aa, synthetic construct
GGEGSDRII

SEQ ID NO: 45110 - protein, 9 aa, synthetic construct
GGEGSDSLN

SEQ ID NO: 45111 - protein, 9 aa, synthetic construct
GGEGSDRIV

SEQ ID NO: 45112 - protein, 9 aa, synthetic construct
GGEGSDRLH

SEQ ID NO: 45113 - protein, 9 aa, synthetic construct
GGEGSDRLL

SEQ ID NO: 45114 - protein, 9 aa, synthetic construct
GGEGSDRLR

SEQ ID NO: 45115 - protein, 9 aa, synthetic construct
GGEGSDRLT

SEQ ID NO: 45116 - protein, 9 aa, synthetic construct
GGEGSDRLW

SEQ ID NO: 45117 - protein, 9 aa, synthetic construct
GGEGSDRMS

SEQ ID NO: 45118 - protein, 9 aa, synthetic construct
GGEGSDRVD

SEQ ID NO: 45119 - protein, 9 aa, synthetic construct
GGEGSDRVE

SEQ ID NO: 45120 - protein, 9 aa, synthetic construct
GGEGSDSAD

SEQ ID NO: 45121 - protein, 9 aa, synthetic construct
GGEGSDSAV

SEQ ID NO: 45122 - protein, 9 aa, synthetic construct
GGEGSDSIF

SEQ ID NO: 45123 - protein, 9 aa, synthetic construct
GGEGSDSII

SEQ ID NO: 45124 - protein, 9 aa, synthetic construct
GGEGSDALH

SEQ ID NO: 45125 - protein, 9 aa, synthetic construct
GGEGSDAIW

SEQ ID NO: 45126 - protein, 9 aa, synthetic construct
GGEGSDAFF

SEQ ID NO: 45127 - protein, 9 aa, synthetic construct
GGEGRDYVY

SEQ ID NO: 45128 - protein, 9 aa, synthetic construct
GGEGRDELY

SEQ ID NO: 45129 - protein, 9 aa, synthetic construct
GGEGRDFIL

SEQ ID NO: 45130 - protein, 9 aa, synthetic construct
GGEGRDFMQ

SEQ ID NO: 45131 - protein, 9 aa, synthetic construct
GGEGRDFVS

SEQ ID NO: 45132 - protein, 9 aa, synthetic construct
GGEGRDGVS

SEQ ID NO: 45133 - protein, 9 aa, synthetic construct
GGEGRDHIL

SEQ ID NO: 45134 - protein, 9 aa, synthetic construct
GGEGRDHLR

SEQ ID NO: 45135 - protein, 9 aa, synthetic construct
GGEGRDIFV

SEQ ID NO: 45136 - protein, 9 aa, synthetic construct
GGEGRDIID

SEQ ID NO: 45137 - protein, 9 aa, synthetic construct
GGEGRDIIE

SEQ ID NO: 45138 - protein, 9 aa, synthetic construct
GGEGRDILA

SEQ ID NO: 45139 - protein, 9 aa, synthetic construct
GGEGRDILK

SEQ ID NO: 45140 - protein, 9 aa, synthetic construct
GGEGRDILL

SEQ ID NO: 45141 - protein, 9 aa, synthetic construct
GGEGRDILN

SEQ ID NO: 45142 - protein, 9 aa, synthetic construct
GGEGRDIMY

SEQ ID NO: 45143 - protein, 9 aa, synthetic construct
GGEGRDIVR

SEQ ID NO: 45144 - protein, 9 aa, synthetic construct
GGEGRDIYN

SEQ ID NO: 45145 - protein, 9 aa, synthetic construct
GGEGRDKLQ

SEQ ID NO: 45146 - protein, 9 aa, synthetic construct
GGEGRDKLS

SEQ ID NO: 45147 - protein, 9 aa, synthetic construct
GGEGRDKLV

SEQ ID NO: 45148 - protein, 9 aa, synthetic construct
GGEGRDKVE

SEQ ID NO: 45149 - protein, 9 aa, synthetic construct
GGEGRDKVY

SEQ ID NO: 45150 - protein, 9 aa, synthetic construct
GGEGRDLLF

SEQ ID NO: 45151 - protein, 9 aa, synthetic construct
GGEGRDLLK

SEQ ID NO: 45152 - protein, 9 aa, synthetic construct
GGEGRDLLL

SEQ ID NO: 45153 - protein, 9 aa, synthetic construct
GGEGRDLLN

SEQ ID NO: 45154 - protein, 9 aa, synthetic construct
GGEGRDLLS

SEQ ID NO: 45155 - protein, 9 aa, synthetic construct
GGEGRDLMS

SEQ ID NO: 45156 - protein, 9 aa, synthetic construct
GGEGRDLVA

SEQ ID NO: 45157 - protein, 9 aa, synthetic construct
GGEGRDELS

SEQ ID NO: 45158 - protein, 9 aa, synthetic construct
GGEGRDELI

SEQ ID NO: 45159 - protein, 9 aa, synthetic construct
GGEGRDELD

SEQ ID NO: 45160 - protein, 9 aa, synthetic construct
GGEGQDVFV

SEQ ID NO: 45161 - protein, 9 aa, synthetic construct
GGEGQDSFV

SEQ ID NO: 45162 - protein, 9 aa, synthetic construct
GGEGQDSIN

SEQ ID NO: 45163 - protein, 9 aa, synthetic construct
GGEGQDSLA

SEQ ID NO: 45164 - protein, 9 aa, synthetic construct
GGEGQDSLF

SEQ ID NO: 45165 - protein, 9 aa, synthetic construct
GGEGQDSLK

SEQ ID NO: 45166 - protein, 9 aa, synthetic construct
GGEGQDSLR

SEQ ID NO: 45167 - protein, 9 aa, synthetic construct
GGEGQDSMR

SEQ ID NO: 45168 - protein, 9 aa, synthetic construct
GGEGQDTAD

SEQ ID NO: 45169 - protein, 9 aa, synthetic construct
GGEGQDTAL

SEQ ID NO: 45170 - protein, 9 aa, synthetic construct
GGEGQDTIT

SEQ ID NO: 45171 - protein, 9 aa, synthetic construct
GGEGQDTLH

SEQ ID NO: 45172 - protein, 9 aa, synthetic construct
GGEGQDTLM

SEQ ID NO: 45173 - protein, 9 aa, synthetic construct
GGEGQDVAM

SEQ ID NO: 45174 - protein, 9 aa, synthetic construct
GGEGQDVLA

SEQ ID NO: 45175 - protein, 9 aa, synthetic construct
GGEGRDEIY

SEQ ID NO: 45176 - protein, 9 aa, synthetic construct
GGEGQDVLR

SEQ ID NO: 45177 - protein, 9 aa, synthetic construct
GGEGQDVVQ

SEQ ID NO: 45178 - protein, 9 aa, synthetic construct
GGEGQDWLA

SEQ ID NO: 45179 - protein, 9 aa, synthetic construct
GGEGRDAFF

SEQ ID NO: 45180 - protein, 9 aa, synthetic construct
GGEGRDAID

SEQ ID NO: 45181 - protein, 9 aa, synthetic construct
GGEGRDAIQ

SEQ ID NO: 45182 - protein, 9 aa, synthetic construct
GGEGRDDFV

SEQ ID NO: 45183 - protein, 9 aa, synthetic construct
GGEGRDDIE

SEQ ID NO: 45184 - protein, 9 aa, synthetic construct
GGEGRDDIS

SEQ ID NO: 45185 - protein, 9 aa, synthetic construct
GGEGRDDIW

SEQ ID NO: 45186 - protein, 9 aa, synthetic construct
GGEGRDDLF

SEQ ID NO: 45187 - protein, 9 aa, synthetic construct
GGEGRDEAH

SEQ ID NO: 45188 - protein, 9 aa, synthetic construct
GGEGRDEIT

SEQ ID NO: 45189 - protein, 9 aa, synthetic construct
GGEGRDLVL

SEQ ID NO: 45190 - protein, 9 aa, synthetic construct
GGEGRDLYL

SEQ ID NO: 45191 - protein, 9 aa, synthetic construct
GGEGRDMFI

SEQ ID NO: 45192 - protein, 9 aa, synthetic construct
GGEGRDTVV

SEQ ID NO: 45193 - protein, 9 aa, synthetic construct
GGEGRDTAR

SEQ ID NO: 45194 - protein, 9 aa, synthetic construct
GGEGRDTAV

SEQ ID NO: 45195 - protein, 9 aa, synthetic construct
GGEGRDTAY

SEQ ID NO: 45196 - protein, 9 aa, synthetic construct
GGEGRDTFI

SEQ ID NO: 45197 - protein, 9 aa, synthetic construct
GGEGRDTFV

SEQ ID NO: 45198 - protein, 9 aa, synthetic construct
GGEGRDTIE

SEQ ID NO: 45199 - protein, 9 aa, synthetic construct
GGEGRDTII

SEQ ID NO: 45200 - protein, 9 aa, synthetic construct
GGEGRDTLQ

SEQ ID NO: 45201 - protein, 9 aa, synthetic construct
GGEGRDTLW

SEQ ID NO: 45202 - protein, 9 aa, synthetic construct
GGEGRDTMA

SEQ ID NO: 45203 - protein, 9 aa, synthetic construct
GGEGRDTMR

SEQ ID NO: 45204 - protein, 9 aa, synthetic construct
GGEGRDTVL

SEQ ID NO: 45205 - protein, 9 aa, synthetic construct
GGEGRDTVQ

SEQ ID NO: 45206 - protein, 9 aa, synthetic construct
GGEGRDTYQ

SEQ ID NO: 45207 - protein, 9 aa, synthetic construct
GGEGRDTAA

SEQ ID NO: 45208 - protein, 9 aa, synthetic construct
GGEGRDVFI

SEQ ID NO: 45209 - protein, 9 aa, synthetic construct
GGEGRDVIT

SEQ ID NO: 45210 - protein, 9 aa, synthetic construct
GGEGRDVIV

SEQ ID NO: 45211 - protein, 9 aa, synthetic construct
GGEGRDVLH

SEQ ID NO: 45212 - protein, 9 aa, synthetic construct
GGEGRDVLN

SEQ ID NO: 45213 - protein, 9 aa, synthetic construct
GGEGRDVMR

SEQ ID NO: 45214 - protein, 9 aa, synthetic construct
GGEGRDVVF

SEQ ID NO: 45215 - protein, 9 aa, synthetic construct
GGEGRDWIE

SEQ ID NO: 45216 - protein, 9 aa, synthetic construct
GGEGRDWIS

SEQ ID NO: 45217 - protein, 9 aa, synthetic construct
GGEGRDWLF

SEQ ID NO: 45218 - protein, 9 aa, synthetic construct
GGEGRDWLW

SEQ ID NO: 45219 - protein, 9 aa, synthetic construct
GGEGRDYID

SEQ ID NO: 45220 - protein, 9 aa, synthetic construct
GGEGRDYLA

SEQ ID NO: 45221 - protein, 9 aa, synthetic construct
GGEGRDTAD

SEQ ID NO: 45222 - protein, 9 aa, synthetic construct
GGEGRDSYD

SEQ ID NO: 45223 - protein, 9 aa, synthetic construct
GGEGRDMIK

SEQ ID NO: 45224 - protein, 9 aa, synthetic construct
GGEGRDRII

SEQ ID NO: 45225 - protein, 9 aa, synthetic construct
GGEGRDNIF

SEQ ID NO: 45226 - protein, 9 aa, synthetic construct
GGEGRDNIG

SEQ ID NO: 45227 - protein, 9 aa, synthetic construct
GGEGRDNLH

SEQ ID NO: 45228 - protein, 9 aa, synthetic construct
GGEGRDNLT

SEQ ID NO: 45229 - protein, 9 aa, synthetic construct
GGEGRDQFV

SEQ ID NO: 45230 - protein, 9 aa, synthetic construct
GGEGRDQLF

SEQ ID NO: 45231 - protein, 9 aa, synthetic construct
GGEGRDQLR

SEQ ID NO: 45232 - protein, 9 aa, synthetic construct
GGEGRDQVD

SEQ ID NO: 45233 - protein, 9 aa, synthetic construct
GGEGRDRAR

SEQ ID NO: 45234 - protein, 9 aa, synthetic construct
GGEGRDRFA

SEQ ID NO: 45235 - protein, 9 aa, synthetic construct
GGEGRDRFV

SEQ ID NO: 45236 - protein, 9 aa, synthetic construct
GGEGRDRFY

SEQ ID NO: 45237 - protein, 9 aa, synthetic construct
GGEGRDRIA

SEQ ID NO: 45238 - protein, 9 aa, synthetic construct
GGEGRDRLE

SEQ ID NO: 45239 - protein, 9 aa, synthetic construct
GGEGRDSVN

SEQ ID NO: 45240 - protein, 9 aa, synthetic construct
GGEGRDRLH

SEQ ID NO: 45241 - protein, 9 aa, synthetic construct
GGEGRDRLL

SEQ ID NO: 45242 - protein, 9 aa, synthetic construct
GGEGRDRLN

SEQ ID NO: 45243 - protein, 9 aa, synthetic construct
GGEGRDRMS

SEQ ID NO: 45244 - protein, 9 aa, synthetic construct
GGEGRDRVY

SEQ ID NO: 45245 - protein, 9 aa, synthetic construct
GGEGRDRYD

SEQ ID NO: 45246 - protein, 9 aa, synthetic construct
GGEGRDSFL

SEQ ID NO: 45247 - protein, 9 aa, synthetic construct
GGEGRDSFR

SEQ ID NO: 45248 - protein, 9 aa, synthetic construct
GGEGRDSFV

SEQ ID NO: 45249 - protein, 9 aa, synthetic construct
GGEGRDSIG

SEQ ID NO: 45250 - protein, 9 aa, synthetic construct
GGEGRDSLK

SEQ ID NO: 45251 - protein, 9 aa, synthetic construct
GGEGRDSLR

SEQ ID NO: 45252 - protein, 9 aa, synthetic construct
GGEGRDSLS

SEQ ID NO: 45253 - protein, 9 aa, synthetic construct
GGEGSDVMD

SEQ ID NO: 45254 - protein, 9 aa, synthetic construct
GGEGSDVMR

SEQ ID NO: 45255 - protein, 9 aa, synthetic construct
GGEGSDVVD

SEQ ID NO: 45256 - protein, 9 aa, synthetic construct
GGEGVDTAN

SEQ ID NO: 45257 - protein, 9 aa, synthetic construct
GGEGXDIVD

SEQ ID NO: 45258 - protein, 9 aa, synthetic construct
GGEGXDQIX

SEQ ID NO: 45259 - protein, 9 aa, synthetic construct
GGEGXDTLR

SEQ ID NO: 45260 - protein, 9 aa, synthetic construct
GGEGXDVLM

SEQ ID NO: 45261 - protein, 9 aa, synthetic construct
GGEGYDALY

SEQ ID NO: 45262 - protein, 9 aa, synthetic construct
GGEGYDGLY

SEQ ID NO: 45263 - protein, 9 aa, synthetic construct
GGEGYDHLY

SEQ ID NO: 45264 - protein, 9 aa, synthetic construct
GGEGYDIAF

SEQ ID NO: 45265 - protein, 9 aa, synthetic construct
GGEGYDIAI

SEQ ID NO: 45266 - protein, 9 aa, synthetic construct
GGEGYDIAS

SEQ ID NO: 45267 - protein, 9 aa, synthetic construct
GGEGYDIIV

SEQ ID NO: 45268 - protein, 9 aa, synthetic construct
GGEGYDILD

SEQ ID NO: 45269 - protein, 9 aa, synthetic construct
GGEGYDIVT

SEQ ID NO: 45270 - protein, 9 aa, synthetic construct
GGEGYDIYI

SEQ ID NO: 45271 - protein, 9 aa, synthetic construct
GGEGYDIYY

SEQ ID NO: 45272 - protein, 9 aa, synthetic construct
GGEGYDKVF

SEQ ID NO: 45273 - protein, 9 aa, synthetic construct
GGEGYDLAS

SEQ ID NO: 45274 - protein, 9 aa, synthetic construct
GGEGYDLIY

SEQ ID NO: 45275 - protein, 9 aa, synthetic construct
GGEGYDLLN

SEQ ID NO: 45276 - protein, 9 aa, synthetic construct
GGEGYDNVT

SEQ ID NO: 45277 - protein, 9 aa, synthetic construct
GGEGYDQLI

SEQ ID NO: 45278 - protein, 9 aa, synthetic construct
GGEGYDRAT

SEQ ID NO: 45279 - protein, 9 aa, synthetic construct
GGEGYDRIT

SEQ ID NO: 45280 - protein, 9 aa, synthetic construct
GGEGYDRLN

SEQ ID NO: 45281 - protein, 9 aa, synthetic construct
GGEGYDRML

SEQ ID NO: 45282 - protein, 9 aa, synthetic construct
GGEGYDTFI

SEQ ID NO: 45283 - protein, 9 aa, synthetic construct
GGEGYDTIN

SEQ ID NO: 45284 - protein, 9 aa, synthetic construct
GGEGYDTIS

SEQ ID NO: 45285 - protein, 9 aa, synthetic construct
GGEGYDTLI

SEQ ID NO: 45286 - protein, 9 aa, synthetic construct
GGEGWDYVS

SEQ ID NO: 45287 - protein, 9 aa, synthetic construct
GGEGWDWIS

SEQ ID NO: 45288 - protein, 9 aa, synthetic construct
GGEGWDVAS

SEQ ID NO: 45289 - protein, 9 aa, synthetic construct
GGEGVDVLL

SEQ ID NO: 45290 - protein, 9 aa, synthetic construct
GGEGVDTIT

SEQ ID NO: 45291 - protein, 9 aa, synthetic construct
GGEGVDTLA

SEQ ID NO: 45292 - protein, 9 aa, synthetic construct
GGEGVDTLI

SEQ ID NO: 45293 - protein, 9 aa, synthetic construct
GGEGVDTLN

SEQ ID NO: 45294 - protein, 9 aa, synthetic construct
GGEGVDTMT

SEQ ID NO: 45295 - protein, 9 aa, synthetic construct
GGEGVDTVV

SEQ ID NO: 45296 - protein, 9 aa, synthetic construct
GGEGVDTYE

SEQ ID NO: 45297 - protein, 9 aa, synthetic construct
GGEGVDVFS

SEQ ID NO: 45298 - protein, 9 aa, synthetic construct
GGEGVDVIE

SEQ ID NO: 45299 - protein, 9 aa, synthetic construct
GGEGVDVIL

SEQ ID NO: 45300 - protein, 9 aa, synthetic construct
GGEGVDVIW

SEQ ID NO: 45301 - protein, 9 aa, synthetic construct
GGEGVDVLA

SEQ ID NO: 45302 - protein, 9 aa, synthetic construct
GGEGVDVLH

SEQ ID NO: 45303 - protein, 9 aa, synthetic construct
GGEGVDVLR

SEQ ID NO: 45304 - protein, 9 aa, synthetic construct
GGEGWDTLY

SEQ ID NO: 45305 - protein, 9 aa, synthetic construct
GGEGVDVYI

SEQ ID NO: 45306 - protein, 9 aa, synthetic construct
GGEGVDWLS

SEQ ID NO: 45307 - protein, 9 aa, synthetic construct
GGEGVDWLY

SEQ ID NO: 45308 - protein, 9 aa, synthetic construct
GGEGVDWVQ

SEQ ID NO: 45309 - protein, 9 aa, synthetic construct
GGEGVDYFY

SEQ ID NO: 45310 - protein, 9 aa, synthetic construct
GGEGVDYLE

SEQ ID NO: 45311 - protein, 9 aa, synthetic construct
GGEGVDYLR

SEQ ID NO: 45312 - protein, 9 aa, synthetic construct
GGEGVDYLY

SEQ ID NO: 45313 - protein, 9 aa, synthetic construct
GGEGWDAVT

SEQ ID NO: 45314 - protein, 9 aa, synthetic construct
GGEGWDILR

SEQ ID NO: 45315 - protein, 9 aa, synthetic construct
GGEGWDLLS

SEQ ID NO: 45316 - protein, 9 aa, synthetic construct
GGEGWDRLD

SEQ ID NO: 45317 - protein, 9 aa, synthetic construct
GGEGWDTID

SEQ ID NO: 45318 - protein, 9 aa, synthetic construct
GGEGYDTLL

SEQ ID NO: 45319 - protein, 9 aa, synthetic construct
GGEGYDTLV

SEQ ID NO: 45320 - protein, 9 aa, synthetic construct
GGEGYDVAQ

SEQ ID NO: 45321 - protein, 9 aa, synthetic construct
GGFGADKLY

SEQ ID NO: 45322 - protein, 9 aa, synthetic construct
GGFGADHFD

SEQ ID NO: 45323 - protein, 9 aa, synthetic construct
GGFGADHFL

SEQ ID NO: 45324 - protein, 9 aa, synthetic construct
GGFGADHLD

SEQ ID NO: 45325 - protein, 9 aa, synthetic construct
GGFGADHLT

SEQ ID NO: 45326 - protein, 9 aa, synthetic construct
GGFGADIFG

SEQ ID NO: 45327 - protein, 9 aa, synthetic construct
GGFGADILH

SEQ ID NO: 45328 - protein, 9 aa, synthetic construct
GGFGADILR

SEQ ID NO: 45329 - protein, 9 aa, synthetic construct
GGFGADILT

SEQ ID NO: 45330 - protein, 9 aa, synthetic construct
GGFGADIMD

SEQ ID NO: 45331 - protein, 9 aa, synthetic construct
GGFGADIMR

SEQ ID NO: 45332 - protein, 9 aa, synthetic construct
GGFGADIMS

SEQ ID NO: 45333 - protein, 9 aa, synthetic construct
GGFGADIVD

SEQ ID NO: 45334 - protein, 9 aa, synthetic construct
GGFGADKLS

SEQ ID NO: 45335 - protein, 9 aa, synthetic construct
GGFGADLIT

SEQ ID NO: 45336 - protein, 9 aa, synthetic construct
GGFGADFLR

SEQ ID NO: 45337 - protein, 9 aa, synthetic construct
GGFGADLLA

SEQ ID NO: 45338 - protein, 9 aa, synthetic construct
GGFGADLLY

SEQ ID NO: 45339 - protein, 9 aa, synthetic construct
GGFGADLVI

SEQ ID NO: 45340 - protein, 9 aa, synthetic construct
GGFGADNID

SEQ ID NO: 45341 - protein, 9 aa, synthetic construct
GGFGADNIE

SEQ ID NO: 45342 - protein, 9 aa, synthetic construct
GGFGADNLK

SEQ ID NO: 45343 - protein, 9 aa, synthetic construct
GGFGADQFT

SEQ ID NO: 45344 - protein, 9 aa, synthetic construct
GGFGADRLL

SEQ ID NO: 45345 - protein, 9 aa, synthetic construct
GGFGADSID

SEQ ID NO: 45346 - protein, 9 aa, synthetic construct
GGFGADSLK

SEQ ID NO: 45347 - protein, 9 aa, synthetic construct
GGFGADSLL

SEQ ID NO: 45348 - protein, 9 aa, synthetic construct
GGFGADSLT

SEQ ID NO: 45349 - protein, 9 aa, synthetic construct
GGFGADSMD

SEQ ID NO: 45350 - protein, 9 aa, synthetic construct
GGFGADGFL

SEQ ID NO: 45351 - protein, 9 aa, synthetic construct
GGFGADFAH

SEQ ID NO: 45352 - protein, 9 aa, synthetic construct
GGEGYDVFS

SEQ ID NO: 45353 - protein, 9 aa, synthetic construct
GGEGYDYMD

SEQ ID NO: 45354 - protein, 9 aa, synthetic construct
GGEGYDVIF

SEQ ID NO: 45355 - protein, 9 aa, synthetic construct
GGEGYDVII

SEQ ID NO: 45356 - protein, 9 aa, synthetic construct
GGEGYDVIR

SEQ ID NO: 45357 - protein, 9 aa, synthetic construct
GGEGYDVLK

SEQ ID NO: 45358 - protein, 9 aa, synthetic construct
GGEGYDVLS

SEQ ID NO: 45359 - protein, 9 aa, synthetic construct
GGEGYDVLY

SEQ ID NO: 45360 - protein, 9 aa, synthetic construct
GGEGYDVMI

SEQ ID NO: 45361 - protein, 9 aa, synthetic construct
GGEGYDVMQ

SEQ ID NO: 45362 - protein, 9 aa, synthetic construct
GGEGYDVMT

SEQ ID NO: 45363 - protein, 9 aa, synthetic construct
GGEGYDVVR

SEQ ID NO: 45364 - protein, 9 aa, synthetic construct
GGEGYDWAS

SEQ ID NO: 45365 - protein, 9 aa, synthetic construct
GGEGYDYAR

SEQ ID NO: 45366 - protein, 9 aa, synthetic construct
GGEGYDYAS

SEQ ID NO: 45367 - protein, 9 aa, synthetic construct
GGFGADAFR

SEQ ID NO: 45368 - protein, 9 aa, synthetic construct
GGFGADEVH

SEQ ID NO: 45369 - protein, 9 aa, synthetic construct
GGFGADAFV

SEQ ID NO: 45370 - protein, 9 aa, synthetic construct
GGFGADALS

SEQ ID NO: 45371 - protein, 9 aa, synthetic construct
GGFGADAMS

SEQ ID NO: 45372 - protein, 9 aa, synthetic construct
GGFGADDLN

SEQ ID NO: 45373 - protein, 9 aa, synthetic construct
GGFGADDLQ

SEQ ID NO: 45374 - protein, 9 aa, synthetic construct
GGFGADDLS

SEQ ID NO: 45375 - protein, 9 aa, synthetic construct
GGFGADDLV

SEQ ID NO: 45376 - protein, 9 aa, synthetic construct
GGFGADEFL

SEQ ID NO: 45377 - protein, 9 aa, synthetic construct
GGFGADEIW

SEQ ID NO: 45378 - protein, 9 aa, synthetic construct
GGFGADELF

SEQ ID NO: 45379 - protein, 9 aa, synthetic construct
GGFGADEMD

SEQ ID NO: 45380 - protein, 9 aa, synthetic construct
GGFGADEMN

SEQ ID NO: 45381 - protein, 9 aa, synthetic construct
GGFGADEVF

SEQ ID NO: 45382 - protein, 9 aa, synthetic construct
GGEGVDTFV

SEQ ID NO: 45383 - protein, 9 aa, synthetic construct
GGEGVDTAE

SEQ ID NO: 45384 - protein, 9 aa, synthetic construct
GGEGSDVYI

SEQ ID NO: 45385 - protein, 9 aa, synthetic construct
GGEGVDSVV

SEQ ID NO: 45386 - protein, 9 aa, synthetic construct
GGEGTDILR

SEQ ID NO: 45387 - protein, 9 aa, synthetic construct
GGEGTDILS

SEQ ID NO: 45388 - protein, 9 aa, synthetic construct
GGEGTDILT

SEQ ID NO: 45389 - protein, 9 aa, synthetic construct
GGEGTDIVE

SEQ ID NO: 45390 - protein, 9 aa, synthetic construct
GGEGTDIYL

SEQ ID NO: 45391 - protein, 9 aa, synthetic construct
GGEGTDKIN

SEQ ID NO: 45392 - protein, 9 aa, synthetic construct
GGEGTDKLD

SEQ ID NO: 45393 - protein, 9 aa, synthetic construct
GGEGTDKLE

SEQ ID NO: 45394 - protein, 9 aa, synthetic construct
GGEGTDKVQ

SEQ ID NO: 45395 - protein, 9 aa, synthetic construct
GGEGTDLAT

SEQ ID NO: 45396 - protein, 9 aa, synthetic construct
GGEGTDLLF

SEQ ID NO: 45397 - protein, 9 aa, synthetic construct
GGEGTDLLS

SEQ ID NO: 45398 - protein, 9 aa, synthetic construct
GGEGTDMAV

SEQ ID NO: 45399 - protein, 9 aa, synthetic construct
GGEGTDMLT

SEQ ID NO: 45400 - protein, 9 aa, synthetic construct
GGEGTDNMT

SEQ ID NO: 45401 - protein, 9 aa, synthetic construct
GGEGTDQAK

SEQ ID NO: 45402 - protein, 9 aa, synthetic construct
GGEGTDQIE

SEQ ID NO: 45403 - protein, 9 aa, synthetic construct
GGEGTDQLL

SEQ ID NO: 45404 - protein, 9 aa, synthetic construct
GGEGTDRLD

SEQ ID NO: 45405 - protein, 9 aa, synthetic construct
GGEGTDRLE

SEQ ID NO: 45406 - protein, 9 aa, synthetic construct
GGEGTDRMI

SEQ ID NO: 45407 - protein, 9 aa, synthetic construct
GGEGTDRMY

SEQ ID NO: 45408 - protein, 9 aa, synthetic construct
GGEGTDRVY

SEQ ID NO: 45409 - protein, 9 aa, synthetic construct
GGEGTDSAV

SEQ ID NO: 45410 - protein, 9 aa, synthetic construct
GGEGTDSID

SEQ ID NO: 45411 - protein, 9 aa, synthetic construct
GGEGTDSLD

SEQ ID NO: 45412 - protein, 9 aa, synthetic construct
GGEGTDSLH

SEQ ID NO: 45413 - protein, 9 aa, synthetic construct
GGEGTDSLS

SEQ ID NO: 45414 - protein, 9 aa, synthetic construct
GGEGTDSLY

SEQ ID NO: 45415 - protein, 9 aa, synthetic construct
GGEGTDILL

SEQ ID NO: 45416 - protein, 9 aa, synthetic construct
GGEGTDILK

SEQ ID NO: 45417 - protein, 9 aa, synthetic construct
GGEGTDILI

SEQ ID NO: 45418 - protein, 9 aa, synthetic construct
GGEGSDYLN

SEQ ID NO: 45419 - protein, 9 aa, synthetic construct
GGEGSDVYL

SEQ ID NO: 45420 - protein, 9 aa, synthetic construct
GGEGSDVYY

SEQ ID NO: 45421 - protein, 9 aa, synthetic construct
GGEGSDWAA

SEQ ID NO: 45422 - protein, 9 aa, synthetic construct
GGEGSDWAV

SEQ ID NO: 45423 - protein, 9 aa, synthetic construct
GGEGSDWLA

SEQ ID NO: 45424 - protein, 9 aa, synthetic construct
GGEGSDWLE

SEQ ID NO: 45425 - protein, 9 aa, synthetic construct
GGEGSDWLT

SEQ ID NO: 45426 - protein, 9 aa, synthetic construct
GGEGSDWME

SEQ ID NO: 45427 - protein, 9 aa, synthetic construct
GGEGSDWVL

SEQ ID NO: 45428 - protein, 9 aa, synthetic construct
GGEGSDYAS

SEQ ID NO: 45429 - protein, 9 aa, synthetic construct
GGEGSDYIE

SEQ ID NO: 45430 - protein, 9 aa, synthetic construct
GGEGSDYIQ

SEQ ID NO: 45431 - protein, 9 aa, synthetic construct
GGEGSDYLE

SEQ ID NO: 45432 - protein, 9 aa, synthetic construct
GGEGSDYLS

SEQ ID NO: 45433 - protein, 9 aa, synthetic construct
GGEGTDILF

SEQ ID NO: 45434 - protein, 9 aa, synthetic construct
GGEGSDYVD

SEQ ID NO: 45435 - protein, 9 aa, synthetic construct
GGEGTDAIT

SEQ ID NO: 45436 - protein, 9 aa, synthetic construct
GGEGTDALN

SEQ ID NO: 45437 - protein, 9 aa, synthetic construct
GGEGTDDMY

SEQ ID NO: 45438 - protein, 9 aa, synthetic construct
GGEGTDEIY

SEQ ID NO: 45439 - protein, 9 aa, synthetic construct
GGEGTDFIV

SEQ ID NO: 45440 - protein, 9 aa, synthetic construct
GGEGTDGLR

SEQ ID NO: 45441 - protein, 9 aa, synthetic construct
GGEGTDHFH

SEQ ID NO: 45442 - protein, 9 aa, synthetic construct
GGEGTDHFV

SEQ ID NO: 45443 - protein, 9 aa, synthetic construct
GGEGTDHLD

SEQ ID NO: 45444 - protein, 9 aa, synthetic construct
GGEGTDHLY

SEQ ID NO: 45445 - protein, 9 aa, synthetic construct
GGEGTDIAD

SEQ ID NO: 45446 - protein, 9 aa, synthetic construct
GGEGTDIID

SEQ ID NO: 45447 - protein, 9 aa, synthetic construct
GGEGTDSVN

SEQ ID NO: 45448 - protein, 9 aa, synthetic construct
GGEGTDTAG

SEQ ID NO: 45449 - protein, 9 aa, synthetic construct
GGEGTDTAH

SEQ ID NO: 45450 - protein, 9 aa, synthetic construct
GGEGVDQIF

SEQ ID NO: 45451 - protein, 9 aa, synthetic construct
GGEGVDLAS

SEQ ID NO: 45452 - protein, 9 aa, synthetic construct
GGEGVDLFS

SEQ ID NO: 45453 - protein, 9 aa, synthetic construct
GGEGVDLFY

SEQ ID NO: 45454 - protein, 9 aa, synthetic construct
GGEGVDLLD

SEQ ID NO: 45455 - protein, 9 aa, synthetic construct
GGEGVDLLI

SEQ ID NO: 45456 - protein, 9 aa, synthetic construct
GGEGVDLLN

SEQ ID NO: 45457 - protein, 9 aa, synthetic construct
GGEGVDLLT

SEQ ID NO: 45458 - protein, 9 aa, synthetic construct
GGEGVDMLY

SEQ ID NO: 45459 - protein, 9 aa, synthetic construct
GGEGVDNID

SEQ ID NO: 45460 - protein, 9 aa, synthetic construct
GGEGVDNLT

SEQ ID NO: 45461 - protein, 9 aa, synthetic construct
GGEGVDNLW

SEQ ID NO: 45462 - protein, 9 aa, synthetic construct
GGEGVDQFY

SEQ ID NO: 45463 - protein, 9 aa, synthetic construct
GGEGVDQID

SEQ ID NO: 45464 - protein, 9 aa, synthetic construct
GGEGVDQMH

SEQ ID NO: 45465 - protein, 9 aa, synthetic construct
GGEGVDKLS

SEQ ID NO: 45466 - protein, 9 aa, synthetic construct
GGEGVDQVD

SEQ ID NO: 45467 - protein, 9 aa, synthetic construct
GGEGVDRAT

SEQ ID NO: 45468 - protein, 9 aa, synthetic construct
GGEGVDRFS

SEQ ID NO: 45469 - protein, 9 aa, synthetic construct
GGEGVDRLE

SEQ ID NO: 45470 - protein, 9 aa, synthetic construct
GGEGVDRLQ

SEQ ID NO: 45471 - protein, 9 aa, synthetic construct
GGEGVDRLR

SEQ ID NO: 45472 - protein, 9 aa, synthetic construct
GGEGVDRMQ

SEQ ID NO: 45473 - protein, 9 aa, synthetic construct
GGEGVDSID

SEQ ID NO: 45474 - protein, 9 aa, synthetic construct
GGEGVDSIE

SEQ ID NO: 45475 - protein, 9 aa, synthetic construct
GGEGVDSIL

SEQ ID NO: 45476 - protein, 9 aa, synthetic construct
GGEGVDSLI

SEQ ID NO: 45477 - protein, 9 aa, synthetic construct
GGEGVDSLR

SEQ ID NO: 45478 - protein, 9 aa, synthetic construct
GGEGVDSLY

SEQ ID NO: 45479 - protein, 9 aa, synthetic construct
GGEGVDKMT

SEQ ID NO: 45480 - protein, 9 aa, synthetic construct
GGEGVDKLK

SEQ ID NO: 45481 - protein, 9 aa, synthetic construct
GGEGTDTLK

SEQ ID NO: 45482 - protein, 9 aa, synthetic construct
GGEGTDYLT

SEQ ID NO: 45483 - protein, 9 aa, synthetic construct
GGEGTDTMT

SEQ ID NO: 45484 - protein, 9 aa, synthetic construct
GGEGTDTVD

SEQ ID NO: 45485 - protein, 9 aa, synthetic construct
GGEGTDTVF

SEQ ID NO: 45486 - protein, 9 aa, synthetic construct
GGEGTDTVT

SEQ ID NO: 45487 - protein, 9 aa, synthetic construct
GGEGTDTVV

SEQ ID NO: 45488 - protein, 9 aa, synthetic construct
GGEGTDVFL

SEQ ID NO: 45489 - protein, 9 aa, synthetic construct
GGEGTDVLN

SEQ ID NO: 45490 - protein, 9 aa, synthetic construct
GGEGTDVLQ

SEQ ID NO: 45491 - protein, 9 aa, synthetic construct
GGEGTDVLR

SEQ ID NO: 45492 - protein, 9 aa, synthetic construct
GGEGTDWFN

SEQ ID NO: 45493 - protein, 9 aa, synthetic construct
GGEGTDYAL

SEQ ID NO: 45494 - protein, 9 aa, synthetic construct
GGEGTDYAV

SEQ ID NO: 45495 - protein, 9 aa, synthetic construct
GGEGTDYFI

SEQ ID NO: 45496 - protein, 9 aa, synthetic construct
GGEGTDYLY

SEQ ID NO: 45497 - protein, 9 aa, synthetic construct
GGEGVDIMN

SEQ ID NO: 45498 - protein, 9 aa, synthetic construct
GGEGVDAAD

SEQ ID NO: 45499 - protein, 9 aa, synthetic construct
GGEGVDALH

SEQ ID NO: 45500 - protein, 9 aa, synthetic construct
GGEGVDAMQ

SEQ ID NO: 45501 - protein, 9 aa, synthetic construct
GGEGVDDIR

SEQ ID NO: 45502 - protein, 9 aa, synthetic construct
GGEGVDELI

SEQ ID NO: 45503 - protein, 9 aa, synthetic construct
GGEGVDEVD

SEQ ID NO: 45504 - protein, 9 aa, synthetic construct
GGEGVDFIA

SEQ ID NO: 45505 - protein, 9 aa, synthetic construct
GGEGVDFIW

SEQ ID NO: 45506 - protein, 9 aa, synthetic construct
GGEGVDFLN

SEQ ID NO: 45507 - protein, 9 aa, synthetic construct
GGEGVDGLY

SEQ ID NO: 45508 - protein, 9 aa, synthetic construct
GGEGVDHAY

SEQ ID NO: 45509 - protein, 9 aa, synthetic construct
GGEGVDIIA

SEQ ID NO: 45510 - protein, 9 aa, synthetic construct
GGEGVDIIH

SEQ ID NO: 45511 - protein, 9 aa, synthetic construct
GGFGVDIIH

SEQ ID NO: 45512 - protein, 9 aa, synthetic construct
GGFGVDIMA

SEQ ID NO: 45513 - protein, 9 aa, synthetic construct
GGGGNDAML

SEQ ID NO: 45514 - protein, 9 aa, synthetic construct
GGGGHDELS

SEQ ID NO: 45515 - protein, 9 aa, synthetic construct
GGGGGDVLF

SEQ ID NO: 45516 - protein, 9 aa, synthetic construct
GGGGGDVLR

SEQ ID NO: 45517 - protein, 9 aa, synthetic construct
GGGGGDVLS

SEQ ID NO: 45518 - protein, 9 aa, synthetic construct
GGGGGDVMD

SEQ ID NO: 45519 - protein, 9 aa, synthetic construct
GGGGGDVMF

SEQ ID NO: 45520 - protein, 9 aa, synthetic construct
GGGGGDVMR

SEQ ID NO: 45521 - protein, 9 aa, synthetic construct
GGGGGDVMS

SEQ ID NO: 45522 - protein, 9 aa, synthetic construct
GGGGGDVVT

SEQ ID NO: 45523 - protein, 9 aa, synthetic construct
GGGGGDWII

SEQ ID NO: 45524 - protein, 9 aa, synthetic construct
GGGGGDYIH

SEQ ID NO: 45525 - protein, 9 aa, synthetic construct
GGGGGDYIV

SEQ ID NO: 45526 - protein, 9 aa, synthetic construct
GGGGGDYLD

SEQ ID NO: 45527 - protein, 9 aa, synthetic construct
GGGGGDYLH

SEQ ID NO: 45528 - protein, 9 aa, synthetic construct
GGGGGDYLL

SEQ ID NO: 45529 - protein, 9 aa, synthetic construct
GGGGGDYLS

SEQ ID NO: 45530 - protein, 9 aa, synthetic construct
GGGGGDYLT

SEQ ID NO: 45531 - protein, 9 aa, synthetic construct
GGGGGDYMN

SEQ ID NO: 45532 - protein, 9 aa, synthetic construct
GGGGGDYVF

SEQ ID NO: 45533 - protein, 9 aa, synthetic construct
GGGGHDAIS

SEQ ID NO: 45534 - protein, 9 aa, synthetic construct
GGGGHDALF

SEQ ID NO: 45535 - protein, 9 aa, synthetic construct
GGGGHDALI

SEQ ID NO: 45536 - protein, 9 aa, synthetic construct
GGGGHDALQ

SEQ ID NO: 45537 - protein, 9 aa, synthetic construct
GGGGHDDIW

SEQ ID NO: 45538 - protein, 9 aa, synthetic construct
GGGGHDDLH

SEQ ID NO: 45539 - protein, 9 aa, synthetic construct
GGGGHDDLS

SEQ ID NO: 45540 - protein, 9 aa, synthetic construct
GGGGHDDLY

SEQ ID NO: 45541 - protein, 9 aa, synthetic construct
GGGGHDDMS

SEQ ID NO: 45542 - protein, 9 aa, synthetic construct
GGGGHDEFT

SEQ ID NO: 45543 - protein, 9 aa, synthetic construct
GGGGHDELH

SEQ ID NO: 45544 - protein, 9 aa, synthetic construct
GGGGGDVLE

SEQ ID NO: 45545 - protein, 9 aa, synthetic construct
GGGGGDVLD

SEQ ID NO: 45546 - protein, 9 aa, synthetic construct
GGGGGDVIF

SEQ ID NO: 45547 - protein, 9 aa, synthetic construct
GGGGGDTFL

SEQ ID NO: 45548 - protein, 9 aa, synthetic construct
GGGGGDRMR

SEQ ID NO: 45549 - protein, 9 aa, synthetic construct
GGGGGDRMT

SEQ ID NO: 45550 - protein, 9 aa, synthetic construct
GGGGGDRYF

SEQ ID NO: 45551 - protein, 9 aa, synthetic construct
GGGGGDSFK

SEQ ID NO: 45552 - protein, 9 aa, synthetic construct
GGGGGDSFL

SEQ ID NO: 45553 - protein, 9 aa, synthetic construct
GGGGGDSID

SEQ ID NO: 45554 - protein, 9 aa, synthetic construct
GGGGGDSII

SEQ ID NO: 45555 - protein, 9 aa, synthetic construct
GGGGGDSLE

SEQ ID NO: 45556 - protein, 9 aa, synthetic construct
GGGGGDSLK

SEQ ID NO: 45557 - protein, 9 aa, synthetic construct
GGGGGDSLR

SEQ ID NO: 45558 - protein, 9 aa, synthetic construct
GGGGGDSYV

SEQ ID NO: 45559 - protein, 9 aa, synthetic construct
GGGGGDTAI

SEQ ID NO: 45560 - protein, 9 aa, synthetic construct
GGGGGDTAM

SEQ ID NO: 45561 - protein, 9 aa, synthetic construct
GGGGGDTFR

SEQ ID NO: 45562 - protein, 9 aa, synthetic construct
GGGGGDVFY

SEQ ID NO: 45563 - protein, 9 aa, synthetic construct
GGGGGDTFS

SEQ ID NO: 45564 - protein, 9 aa, synthetic construct
GGGGGDTIL

SEQ ID NO: 45565 - protein, 9 aa, synthetic construct
GGGGGDTIN

SEQ ID NO: 45566 - protein, 9 aa, synthetic construct
GGGGGDTIR

SEQ ID NO: 45567 - protein, 9 aa, synthetic construct
GGGGGDTMI

SEQ ID NO: 45568 - protein, 9 aa, synthetic construct
GGGGGDTMN

SEQ ID NO: 45569 - protein, 9 aa, synthetic construct
GGGGGDTMT

SEQ ID NO: 45570 - protein, 9 aa, synthetic construct
GGGGGDTMV

SEQ ID NO: 45571 - protein, 9 aa, synthetic construct
GGGGGDTVS

SEQ ID NO: 45572 - protein, 9 aa, synthetic construct
GGGGGDTYQ

SEQ ID NO: 45573 - protein, 9 aa, synthetic construct
GGGGGDVAR

SEQ ID NO: 45574 - protein, 9 aa, synthetic construct
GGGGGDVFD

SEQ ID NO: 45575 - protein, 9 aa, synthetic construct
GGGGGDVFK

SEQ ID NO: 45576 - protein, 9 aa, synthetic construct
GGGGHDELN

SEQ ID NO: 45577 - protein, 9 aa, synthetic construct
GGGGHDELW

SEQ ID NO: 45578 - protein, 9 aa, synthetic construct
GGGGHDTMN

SEQ ID NO: 45579 - protein, 9 aa, synthetic construct
GGGGHDEMH

SEQ ID NO: 45580 - protein, 9 aa, synthetic construct
GGGGHDQLF

SEQ ID NO: 45581 - protein, 9 aa, synthetic construct
GGGGHDQLG

SEQ ID NO: 45582 - protein, 9 aa, synthetic construct
GGGGHDQLS

SEQ ID NO: 45583 - protein, 9 aa, synthetic construct
GGGGHDRFV

SEQ ID NO: 45584 - protein, 9 aa, synthetic construct
GGGGHDRIV

SEQ ID NO: 45585 - protein, 9 aa, synthetic construct
GGGGHDRIY

SEQ ID NO: 45586 - protein, 9 aa, synthetic construct
GGGGHDRLA

SEQ ID NO: 45587 - protein, 9 aa, synthetic construct
GGGGHDRLW

SEQ ID NO: 45588 - protein, 9 aa, synthetic construct
GGGGHDRMQ

SEQ ID NO: 45589 - protein, 9 aa, synthetic construct
GGGGHDRMT

SEQ ID NO: 45590 - protein, 9 aa, synthetic construct
GGGGHDRYV

SEQ ID NO: 45591 - protein, 9 aa, synthetic construct
GGGGHDRYY

SEQ ID NO: 45592 - protein, 9 aa, synthetic construct
GGGGHDSFL

SEQ ID NO: 45593 - protein, 9 aa, synthetic construct
GGGGHDSIL

SEQ ID NO: 45594 - protein, 9 aa, synthetic construct
GGGGHDSIN

SEQ ID NO: 45595 - protein, 9 aa, synthetic construct
GGGGHDSIV

SEQ ID NO: 45596 - protein, 9 aa, synthetic construct
GGGGHDSLG

SEQ ID NO: 45597 - protein, 9 aa, synthetic construct
GGGGHDSLN

SEQ ID NO: 45598 - protein, 9 aa, synthetic construct
GGGGHDSLT

SEQ ID NO: 45599 - protein, 9 aa, synthetic construct
GGGGHDSLY

SEQ ID NO: 45600 - protein, 9 aa, synthetic construct
GGGGHDSVE

SEQ ID NO: 45601 - protein, 9 aa, synthetic construct
GGGGHDTAI

SEQ ID NO: 45602 - protein, 9 aa, synthetic construct
GGGGHDTID

SEQ ID NO: 45603 - protein, 9 aa, synthetic construct
GGGGHDTIF

SEQ ID NO: 45604 - protein, 9 aa, synthetic construct
GGGGHDTIH

SEQ ID NO: 45605 - protein, 9 aa, synthetic construct
GGGGHDTIS

SEQ ID NO: 45606 - protein, 9 aa, synthetic construct
GGGGHDTIY

SEQ ID NO: 45607 - protein, 9 aa, synthetic construct
GGGGHDTLF

SEQ ID NO: 45608 - protein, 9 aa, synthetic construct
GGGGHDTLM

SEQ ID NO: 45609 - protein, 9 aa, synthetic construct
GGGGHDQLD

SEQ ID NO: 45610 - protein, 9 aa, synthetic construct
GGGGHDNYY

SEQ ID NO: 45611 - protein, 9 aa, synthetic construct
GGGGHDNLA

SEQ ID NO: 45612 - protein, 9 aa, synthetic construct
GGGGHDILR

SEQ ID NO: 45613 - protein, 9 aa, synthetic construct
GGGGHDEMR

SEQ ID NO: 45614 - protein, 9 aa, synthetic construct
GGGGHDFIT

SEQ ID NO: 45615 - protein, 9 aa, synthetic construct
GGGGHDFLV

SEQ ID NO: 45616 - protein, 9 aa, synthetic construct
GGGGHDFVW

SEQ ID NO: 45617 - protein, 9 aa, synthetic construct
GGGGHDGLD

SEQ ID NO: 45618 - protein, 9 aa, synthetic construct
GGGGHDHLE

SEQ ID NO: 45619 - protein, 9 aa, synthetic construct
GGGGHDHLF

SEQ ID NO: 45620 - protein, 9 aa, synthetic construct
GGGGHDHLI

SEQ ID NO: 45621 - protein, 9 aa, synthetic construct
GGGGHDHLS

SEQ ID NO: 45622 - protein, 9 aa, synthetic construct
GGGGHDIID

SEQ ID NO: 45623 - protein, 9 aa, synthetic construct
GGGGHDIIV

SEQ ID NO: 45624 - protein, 9 aa, synthetic construct
GGGGHDILE

SEQ ID NO: 45625 - protein, 9 aa, synthetic construct
GGGGHDILL

SEQ ID NO: 45626 - protein, 9 aa, synthetic construct
GGGGHDIMD

SEQ ID NO: 45627 - protein, 9 aa, synthetic construct
GGGGHDNID

SEQ ID NO: 45628 - protein, 9 aa, synthetic construct
GGGGHDKLD

SEQ ID NO: 45629 - protein, 9 aa, synthetic construct
GGGGHDKLF

SEQ ID NO: 45630 - protein, 9 aa, synthetic construct
GGGGHDKLS

SEQ ID NO: 45631 - protein, 9 aa, synthetic construct
GGGGHDLFW

SEQ ID NO: 45632 - protein, 9 aa, synthetic construct
GGGGHDLIF

SEQ ID NO: 45633 - protein, 9 aa, synthetic construct
GGGGHDLLF

SEQ ID NO: 45634 - protein, 9 aa, synthetic construct
GGGGHDLLI

SEQ ID NO: 45635 - protein, 9 aa, synthetic construct
GGGGHDLLL

SEQ ID NO: 45636 - protein, 9 aa, synthetic construct
GGGGHDLLQ

SEQ ID NO: 45637 - protein, 9 aa, synthetic construct
GGGGHDLLR

SEQ ID NO: 45638 - protein, 9 aa, synthetic construct
GGGGHDLMF

SEQ ID NO: 45639 - protein, 9 aa, synthetic construct
GGGGHDLMN

SEQ ID NO: 45640 - protein, 9 aa, synthetic construct
GGGGHDMLN

SEQ ID NO: 45641 - protein, 9 aa, synthetic construct
GGGGGDRMD

SEQ ID NO: 45642 - protein, 9 aa, synthetic construct
GGGGGDRLR

SEQ ID NO: 45643 - protein, 9 aa, synthetic construct
GGGGGDRLQ

SEQ ID NO: 45644 - protein, 9 aa, synthetic construct
GGGGGDRLN

SEQ ID NO: 45645 - protein, 9 aa, synthetic construct
GGGGFDILT

SEQ ID NO: 45646 - protein, 9 aa, synthetic construct
GGGGFDKFF

SEQ ID NO: 45647 - protein, 9 aa, synthetic construct
GGGGFDLFG

SEQ ID NO: 45648 - protein, 9 aa, synthetic construct
GGGGFDLLS

SEQ ID NO: 45649 - protein, 9 aa, synthetic construct
GGGGFDLLY

SEQ ID NO: 45650 - protein, 9 aa, synthetic construct
GGGGFDNFI

SEQ ID NO: 45651 - protein, 9 aa, synthetic construct
GGGGFDNIF

SEQ ID NO: 45652 - protein, 9 aa, synthetic construct
GGGGFDRFI

SEQ ID NO: 45653 - protein, 9 aa, synthetic construct
GGGGFDRLE

SEQ ID NO: 45654 - protein, 9 aa, synthetic construct
GGGGFDRLS

SEQ ID NO: 45655 - protein, 9 aa, synthetic construct
GGGGFDSIF

SEQ ID NO: 45656 - protein, 9 aa, synthetic construct
GGGGFDSIL

SEQ ID NO: 45657 - protein, 9 aa, synthetic construct
GGGGFDSLW

SEQ ID NO: 45658 - protein, 9 aa, synthetic construct
GGGGFDSVV

SEQ ID NO: 45659 - protein, 9 aa, synthetic construct
GGGGFDTFD

SEQ ID NO: 45660 - protein, 9 aa, synthetic construct
GGGGFDTFT

SEQ ID NO: 45661 - protein, 9 aa, synthetic construct
GGGGFDTLD

SEQ ID NO: 45662 - protein, 9 aa, synthetic construct
GGGGFDTLF

SEQ ID NO: 45663 - protein, 9 aa, synthetic construct
GGGGFDTMR

SEQ ID NO: 45664 - protein, 9 aa, synthetic construct
GGGGFDTVY

SEQ ID NO: 45665 - protein, 9 aa, synthetic construct
GGGGFDVLI

SEQ ID NO: 45666 - protein, 9 aa, synthetic construct
GGGGFDVLN

SEQ ID NO: 45667 - protein, 9 aa, synthetic construct
GGGGFDVVF

SEQ ID NO: 45668 - protein, 9 aa, synthetic construct
GGGGFDVVS

SEQ ID NO: 45669 - protein, 9 aa, synthetic construct
GGGGFDWAS

SEQ ID NO: 45670 - protein, 9 aa, synthetic construct
GGGGFDYAD

SEQ ID NO: 45671 - protein, 9 aa, synthetic construct
GGGGGDAFR

SEQ ID NO: 45672 - protein, 9 aa, synthetic construct
GGGGGDAFV

SEQ ID NO: 45673 - protein, 9 aa, synthetic construct
GGGGGDAID

SEQ ID NO: 45674 - protein, 9 aa, synthetic construct
GGGGFDILS

SEQ ID NO: 45675 - protein, 9 aa, synthetic construct
GGGGFDILD

SEQ ID NO: 45676 - protein, 9 aa, synthetic construct
GGGGFDIIV

SEQ ID NO: 45677 - protein, 9 aa, synthetic construct
GGGGEDVLL

SEQ ID NO: 45678 - protein, 9 aa, synthetic construct
GGGGEDSVV

SEQ ID NO: 45679 - protein, 9 aa, synthetic construct
GGGGEDTFR

SEQ ID NO: 45680 - protein, 9 aa, synthetic construct
GGGGEDTIG

SEQ ID NO: 45681 - protein, 9 aa, synthetic construct
GGGGEDTIH

SEQ ID NO: 45682 - protein, 9 aa, synthetic construct
GGGGEDTLD

SEQ ID NO: 45683 - protein, 9 aa, synthetic construct
GGGGEDTLQ

SEQ ID NO: 45684 - protein, 9 aa, synthetic construct
GGGGEDTLR

SEQ ID NO: 45685 - protein, 9 aa, synthetic construct
GGGGEDTVF

SEQ ID NO: 45686 - protein, 9 aa, synthetic construct
GGGGEDTVY

SEQ ID NO: 45687 - protein, 9 aa, synthetic construct
GGGGEDTYV

SEQ ID NO: 45688 - protein, 9 aa, synthetic construct
GGGGEDVFK

SEQ ID NO: 45689 - protein, 9 aa, synthetic construct
GGGGEDVFR

SEQ ID NO: 45690 - protein, 9 aa, synthetic construct
GGGGEDVLI

SEQ ID NO: 45691 - protein, 9 aa, synthetic construct
GGGGEDVLN

SEQ ID NO: 45692 - protein, 9 aa, synthetic construct
GGGGFDIAD

SEQ ID NO: 45693 - protein, 9 aa, synthetic construct
GGGGEDVLS

SEQ ID NO: 45694 - protein, 9 aa, synthetic construct
GGGGEDVLY

SEQ ID NO: 45695 - protein, 9 aa, synthetic construct
GGGGEDVMT

SEQ ID NO: 45696 - protein, 9 aa, synthetic construct
GGGGEDWAA

SEQ ID NO: 45697 - protein, 9 aa, synthetic construct
GGGGEDWLF

SEQ ID NO: 45698 - protein, 9 aa, synthetic construct
GGGGEDYLY

SEQ ID NO: 45699 - protein, 9 aa, synthetic construct
GGGGFDAMA

SEQ ID NO: 45700 - protein, 9 aa, synthetic construct
GGGGFDDAG

SEQ ID NO: 45701 - protein, 9 aa, synthetic construct
GGGGFDDIN

SEQ ID NO: 45702 - protein, 9 aa, synthetic construct
GGGGFDEAT

SEQ ID NO: 45703 - protein, 9 aa, synthetic construct
GGGGFDEVN

SEQ ID NO: 45704 - protein, 9 aa, synthetic construct
GGGGFDFLD

SEQ ID NO: 45705 - protein, 9 aa, synthetic construct
GGGGFDHLS

SEQ ID NO: 45706 - protein, 9 aa, synthetic construct
GGGGGDALA

SEQ ID NO: 45707 - protein, 9 aa, synthetic construct
GGGGGDALT

SEQ ID NO: 45708 - protein, 9 aa, synthetic construct
GGGGGDDAG

SEQ ID NO: 45709 - protein, 9 aa, synthetic construct
GGGGGDQIK

SEQ ID NO: 45710 - protein, 9 aa, synthetic construct
GGGGGDLLL

SEQ ID NO: 45711 - protein, 9 aa, synthetic construct
GGGGGDLLQ

SEQ ID NO: 45712 - protein, 9 aa, synthetic construct
GGGGGDLLS

SEQ ID NO: 45713 - protein, 9 aa, synthetic construct
GGGGGDLLV

SEQ ID NO: 45714 - protein, 9 aa, synthetic construct
GGGGGDLMT

SEQ ID NO: 45715 - protein, 9 aa, synthetic construct
GGGGGDLVF

SEQ ID NO: 45716 - protein, 9 aa, synthetic construct
GGGGGDLVL

SEQ ID NO: 45717 - protein, 9 aa, synthetic construct
GGGGGDMFS

SEQ ID NO: 45718 - protein, 9 aa, synthetic construct
GGGGGDMLT

SEQ ID NO: 45719 - protein, 9 aa, synthetic construct
GGGGGDNLD

SEQ ID NO: 45720 - protein, 9 aa, synthetic construct
GGGGGDNLF

SEQ ID NO: 45721 - protein, 9 aa, synthetic construct
GGGGGDNLN

SEQ ID NO: 45722 - protein, 9 aa, synthetic construct
GGGGGDQIF

SEQ ID NO: 45723 - protein, 9 aa, synthetic construct
GGGGGDQIN

SEQ ID NO: 45724 - protein, 9 aa, synthetic construct
GGGGGDLLE

SEQ ID NO: 45725 - protein, 9 aa, synthetic construct
GGGGGDQIS

SEQ ID NO: 45726 - protein, 9 aa, synthetic construct
GGGGGDQIV

SEQ ID NO: 45727 - protein, 9 aa, synthetic construct
GGGGGDQLD

SEQ ID NO: 45728 - protein, 9 aa, synthetic construct
GGGGGDQLS

SEQ ID NO: 45729 - protein, 9 aa, synthetic construct
GGGGGDQLW

SEQ ID NO: 45730 - protein, 9 aa, synthetic construct
GGGGGDQML

SEQ ID NO: 45731 - protein, 9 aa, synthetic construct
GGGGGDQVL

SEQ ID NO: 45732 - protein, 9 aa, synthetic construct
GGGGGDRFA

SEQ ID NO: 45733 - protein, 9 aa, synthetic construct
GGGGGDRII

SEQ ID NO: 45734 - protein, 9 aa, synthetic construct
GGGGGDRIV

SEQ ID NO: 45735 - protein, 9 aa, synthetic construct
GGGGGDRLF

SEQ ID NO: 45736 - protein, 9 aa, synthetic construct
GGGGGDRLH

SEQ ID NO: 45737 - protein, 9 aa, synthetic construct
GGGGGDRLK

SEQ ID NO: 45738 - protein, 9 aa, synthetic construct
GGGGGDLLH

SEQ ID NO: 45739 - protein, 9 aa, synthetic construct
GGGGGDLLA

SEQ ID NO: 45740 - protein, 9 aa, synthetic construct
GGGGGDDAT

SEQ ID NO: 45741 - protein, 9 aa, synthetic construct
GGGGGDGLF

SEQ ID NO: 45742 - protein, 9 aa, synthetic construct
GGGGGDDFY

SEQ ID NO: 45743 - protein, 9 aa, synthetic construct
GGGGGDDLH

SEQ ID NO: 45744 - protein, 9 aa, synthetic construct
GGGGGDDLQ

SEQ ID NO: 45745 - protein, 9 aa, synthetic construct
GGGGGDDLS

SEQ ID NO: 45746 - protein, 9 aa, synthetic construct
GGGGGDDLY

SEQ ID NO: 45747 - protein, 9 aa, synthetic construct
GGGGGDDMR

SEQ ID NO: 45748 - protein, 9 aa, synthetic construct
GGGGGDDVD

SEQ ID NO: 45749 - protein, 9 aa, synthetic construct
GGGGGDEAS

SEQ ID NO: 45750 - protein, 9 aa, synthetic construct
GGGGGDEIT

SEQ ID NO: 45751 - protein, 9 aa, synthetic construct
GGGGGDELL

SEQ ID NO: 45752 - protein, 9 aa, synthetic construct
GGGGGDELS

SEQ ID NO: 45753 - protein, 9 aa, synthetic construct
GGGGGDFVN

SEQ ID NO: 45754 - protein, 9 aa, synthetic construct
GGGGGDGFR

SEQ ID NO: 45755 - protein, 9 aa, synthetic construct
GGGGGDGLN

SEQ ID NO: 45756 - protein, 9 aa, synthetic construct
GGGGGDLIS

SEQ ID NO: 45757 - protein, 9 aa, synthetic construct
GGGGGDHIY

SEQ ID NO: 45758 - protein, 9 aa, synthetic construct
GGGGGDIID

SEQ ID NO: 45759 - protein, 9 aa, synthetic construct
GGGGGDIII

SEQ ID NO: 45760 - protein, 9 aa, synthetic construct
GGGGGDIIS

SEQ ID NO: 45761 - protein, 9 aa, synthetic construct
GGGGGDILD

SEQ ID NO: 45762 - protein, 9 aa, synthetic construct
GGGGGDILI

SEQ ID NO: 45763 - protein, 9 aa, synthetic construct
GGGGGDIMK

SEQ ID NO: 45764 - protein, 9 aa, synthetic construct
GGGGGDKLK

SEQ ID NO: 45765 - protein, 9 aa, synthetic construct
GGGGGDKLR

SEQ ID NO: 45766 - protein, 9 aa, synthetic construct
GGGGGDKMR

SEQ ID NO: 45767 - protein, 9 aa, synthetic construct
GGGGGDLFY

SEQ ID NO: 45768 - protein, 9 aa, synthetic construct
GGGGGDLID

SEQ ID NO: 45769 - protein, 9 aa, synthetic construct
GGGGGDLIF

SEQ ID NO: 45770 - protein, 9 aa, synthetic construct
GGGGHDTMD

SEQ ID NO: 45771 - protein, 9 aa, synthetic construct
GGGGHDTMQ

SEQ ID NO: 45772 - protein, 9 aa, synthetic construct
GGFGVDIVI

SEQ ID NO: 45773 - protein, 9 aa, synthetic construct
GGGGLDLLN

SEQ ID NO: 45774 - protein, 9 aa, synthetic construct
GGGGKDVAS

SEQ ID NO: 45775 - protein, 9 aa, synthetic construct
GGGGKDVFY

SEQ ID NO: 45776 - protein, 9 aa, synthetic construct
GGGGKDVIN

SEQ ID NO: 45777 - protein, 9 aa, synthetic construct
GGGGKDVIY

SEQ ID NO: 45778 - protein, 9 aa, synthetic construct
GGGGKDVLF

SEQ ID NO: 45779 - protein, 9 aa, synthetic construct
GGGGKDVLI

SEQ ID NO: 45780 - protein, 9 aa, synthetic construct
GGGGKDVLM

SEQ ID NO: 45781 - protein, 9 aa, synthetic construct
GGGGKDVLN

SEQ ID NO: 45782 - protein, 9 aa, synthetic construct
GGGGKDVLQ

SEQ ID NO: 45783 - protein, 9 aa, synthetic construct
GGGGKDVMI

SEQ ID NO: 45784 - protein, 9 aa, synthetic construct
GGGGKDVVF

SEQ ID NO: 45785 - protein, 9 aa, synthetic construct
GGGGKDYFE

SEQ ID NO: 45786 - protein, 9 aa, synthetic construct
GGGGKDYLQ

SEQ ID NO: 45787 - protein, 9 aa, synthetic construct
GGGGKDYLY

SEQ ID NO: 45788 - protein, 9 aa, synthetic construct
GGGGLDAIY

SEQ ID NO: 45789 - protein, 9 aa, synthetic construct
GGGGLDAMI

SEQ ID NO: 45790 - protein, 9 aa, synthetic construct
GGGGLDDLY

SEQ ID NO: 45791 - protein, 9 aa, synthetic construct
GGGGLDEFF

SEQ ID NO: 45792 - protein, 9 aa, synthetic construct
GGGGLDELV

SEQ ID NO: 45793 - protein, 9 aa, synthetic construct
GGGGLDEMH

SEQ ID NO: 45794 - protein, 9 aa, synthetic construct
GGGGLDHLF

SEQ ID NO: 45795 - protein, 9 aa, synthetic construct
GGGGLDIFR

SEQ ID NO: 45796 - protein, 9 aa, synthetic construct
GGGGLDIIS

SEQ ID NO: 45797 - protein, 9 aa, synthetic construct
GGGGLDILF

SEQ ID NO: 45798 - protein, 9 aa, synthetic construct
GGGGLDILM

SEQ ID NO: 45799 - protein, 9 aa, synthetic construct
GGGGLDILS

SEQ ID NO: 45800 - protein, 9 aa, synthetic construct
GGGGLDILT

SEQ ID NO: 45801 - protein, 9 aa, synthetic construct
GGGGLDIVN

SEQ ID NO: 45802 - protein, 9 aa, synthetic construct
GGGGLDKLF

SEQ ID NO: 45803 - protein, 9 aa, synthetic construct
GGGGKDTYV

SEQ ID NO: 45804 - protein, 9 aa, synthetic construct
GGGGKDTVY

SEQ ID NO: 45805 - protein, 9 aa, synthetic construct
GGGGKDTVS

SEQ ID NO: 45806 - protein, 9 aa, synthetic construct
GGGGKDSLE

SEQ ID NO: 45807 - protein, 9 aa, synthetic construct
GGGGKDQLF

SEQ ID NO: 45808 - protein, 9 aa, synthetic construct
GGGGKDQLM

SEQ ID NO: 45809 - protein, 9 aa, synthetic construct
GGGGKDQLN

SEQ ID NO: 45810 - protein, 9 aa, synthetic construct
GGGGKDQVY

SEQ ID NO: 45811 - protein, 9 aa, synthetic construct
GGGGKDRFD

SEQ ID NO: 45812 - protein, 9 aa, synthetic construct
GGGGKDRFI

SEQ ID NO: 45813 - protein, 9 aa, synthetic construct
GGGGKDRIA

SEQ ID NO: 45814 - protein, 9 aa, synthetic construct
GGGGKDRLE

SEQ ID NO: 45815 - protein, 9 aa, synthetic construct
GGGGKDRLF

SEQ ID NO: 45816 - protein, 9 aa, synthetic construct
GGGGKDRLV

SEQ ID NO: 45817 - protein, 9 aa, synthetic construct
GGGGKDRLW

SEQ ID NO: 45818 - protein, 9 aa, synthetic construct
GGGGKDSFV

SEQ ID NO: 45819 - protein, 9 aa, synthetic construct
GGGGKDSIY

SEQ ID NO: 45820 - protein, 9 aa, synthetic construct
GGGGKDSLG

SEQ ID NO: 45821 - protein, 9 aa, synthetic construct
GGGGKDTVL

SEQ ID NO: 45822 - protein, 9 aa, synthetic construct
GGGGKDSLK

SEQ ID NO: 45823 - protein, 9 aa, synthetic construct
GGGGKDSLR

SEQ ID NO: 45824 - protein, 9 aa, synthetic construct
GGGGKDSLS

SEQ ID NO: 45825 - protein, 9 aa, synthetic construct
GGGGKDSLV

SEQ ID NO: 45826 - protein, 9 aa, synthetic construct
GGGGKDSLY

SEQ ID NO: 45827 - protein, 9 aa, synthetic construct
GGGGKDSMQ

SEQ ID NO: 45828 - protein, 9 aa, synthetic construct
GGGGKDTAR

SEQ ID NO: 45829 - protein, 9 aa, synthetic construct
GGGGKDTFQ

SEQ ID NO: 45830 - protein, 9 aa, synthetic construct
GGGGKDTLA

SEQ ID NO: 45831 - protein, 9 aa, synthetic construct
GGGGKDTLE

SEQ ID NO: 45832 - protein, 9 aa, synthetic construct
GGGGKDTLM

SEQ ID NO: 45833 - protein, 9 aa, synthetic construct
GGGGKDTLR

SEQ ID NO: 45834 - protein, 9 aa, synthetic construct
GGGGKDTLY

SEQ ID NO: 45835 - protein, 9 aa, synthetic construct
GGGGLDLLK

SEQ ID NO: 45836 - protein, 9 aa, synthetic construct
GGGGLDLLY

SEQ ID NO: 45837 - protein, 9 aa, synthetic construct
GGGGHDTMY

SEQ ID NO: 45838 - protein, 9 aa, synthetic construct
GGGGLDNLY

SEQ ID NO: 45839 - protein, 9 aa, synthetic construct
GGGGLDVLR

SEQ ID NO: 45840 - protein, 9 aa, synthetic construct
GGGGLDVLY

SEQ ID NO: 45841 - protein, 9 aa, synthetic construct
GGGGLDVMS

SEQ ID NO: 45842 - protein, 9 aa, synthetic construct
GGGGLDYLD

SEQ ID NO: 45843 - protein, 9 aa, synthetic construct
GGGGMDCLT

SEQ ID NO: 45844 - protein, 9 aa, synthetic construct
GGGGMDEMY

SEQ ID NO: 45845 - protein, 9 aa, synthetic construct
GGGGMDFYV

SEQ ID NO: 45846 - protein, 9 aa, synthetic construct
GGGGMDGVS

SEQ ID NO: 45847 - protein, 9 aa, synthetic construct
GGGGMDIFA

SEQ ID NO: 45848 - protein, 9 aa, synthetic construct
GGGGMDILT

SEQ ID NO: 45849 - protein, 9 aa, synthetic construct
GGGGMDLVN

SEQ ID NO: 45850 - protein, 9 aa, synthetic construct
GGGGMDTAD

SEQ ID NO: 45851 - protein, 9 aa, synthetic construct
GGGGMDTFN

SEQ ID NO: 45852 - protein, 9 aa, synthetic construct
GGGGMDTLT

SEQ ID NO: 45853 - protein, 9 aa, synthetic construct
GGGGMDTVQ

SEQ ID NO: 45854 - protein, 9 aa, synthetic construct
GGGGMDTVS

SEQ ID NO: 45855 - protein, 9 aa, synthetic construct
GGGGMDVIS

SEQ ID NO: 45856 - protein, 9 aa, synthetic construct
GGGGMDVLI

SEQ ID NO: 45857 - protein, 9 aa, synthetic construct
GGGGMDVLY

SEQ ID NO: 45858 - protein, 9 aa, synthetic construct
GGGGMDWIE

SEQ ID NO: 45859 - protein, 9 aa, synthetic construct
GGGGMDWLD

SEQ ID NO: 45860 - protein, 9 aa, synthetic construct
GGGGMDYAD

SEQ ID NO: 45861 - protein, 9 aa, synthetic construct
GGGGNDAFY

SEQ ID NO: 45862 - protein, 9 aa, synthetic construct
GGGGNDAIF

SEQ ID NO: 45863 - protein, 9 aa, synthetic construct
GGGGNDAIH

SEQ ID NO: 45864 - protein, 9 aa, synthetic construct
GGGGNDALK

SEQ ID NO: 45865 - protein, 9 aa, synthetic construct
GGGGNDALL

SEQ ID NO: 45866 - protein, 9 aa, synthetic construct
GGGGNDALQ

SEQ ID NO: 45867 - protein, 9 aa, synthetic construct
GGGGNDAMD

SEQ ID NO: 45868 - protein, 9 aa, synthetic construct
GGGGLDVLQ

SEQ ID NO: 45869 - protein, 9 aa, synthetic construct
GGGGLDVLH

SEQ ID NO: 45870 - protein, 9 aa, synthetic construct
GGGGLDVFN

SEQ ID NO: 45871 - protein, 9 aa, synthetic construct
GGGGLDTAD

SEQ ID NO: 45872 - protein, 9 aa, synthetic construct
GGGGLDQLF

SEQ ID NO: 45873 - protein, 9 aa, synthetic construct
GGGGLDQLL

SEQ ID NO: 45874 - protein, 9 aa, synthetic construct
GGGGLDQLS

SEQ ID NO: 45875 - protein, 9 aa, synthetic construct
GGGGLDQLT

SEQ ID NO: 45876 - protein, 9 aa, synthetic construct
GGGGLDRIE

SEQ ID NO: 45877 - protein, 9 aa, synthetic construct
GGGGLDRIN

SEQ ID NO: 45878 - protein, 9 aa, synthetic construct
GGGGLDRLA

SEQ ID NO: 45879 - protein, 9 aa, synthetic construct
GGGGLDRLN

SEQ ID NO: 45880 - protein, 9 aa, synthetic construct
GGGGLDSFG

SEQ ID NO: 45881 - protein, 9 aa, synthetic construct
GGGGLDSIN

SEQ ID NO: 45882 - protein, 9 aa, synthetic construct
GGGGLDSLD

SEQ ID NO: 45883 - protein, 9 aa, synthetic construct
GGGGLDSLL

SEQ ID NO: 45884 - protein, 9 aa, synthetic construct
GGGGLDSLY

SEQ ID NO: 45885 - protein, 9 aa, synthetic construct
GGGGLDTAL

SEQ ID NO: 45886 - protein, 9 aa, synthetic construct
GGGGLDVFH

SEQ ID NO: 45887 - protein, 9 aa, synthetic construct
GGGGLDTIF

SEQ ID NO: 45888 - protein, 9 aa, synthetic construct
GGGGLDTIL

SEQ ID NO: 45889 - protein, 9 aa, synthetic construct
GGGGLDTLA

SEQ ID NO: 45890 - protein, 9 aa, synthetic construct
GGGGLDTLE

SEQ ID NO: 45891 - protein, 9 aa, synthetic construct
GGGGLDTLF

SEQ ID NO: 45892 - protein, 9 aa, synthetic construct
GGGGLDTLL

SEQ ID NO: 45893 - protein, 9 aa, synthetic construct
GGGGLDTLM

SEQ ID NO: 45894 - protein, 9 aa, synthetic construct
GGGGLDTLQ

SEQ ID NO: 45895 - protein, 9 aa, synthetic construct
GGGGLDTLR

SEQ ID NO: 45896 - protein, 9 aa, synthetic construct
GGGGLDTLS

SEQ ID NO: 45897 - protein, 9 aa, synthetic construct
GGGGLDTLT

SEQ ID NO: 45898 - protein, 9 aa, synthetic construct
GGGGLDTMN

SEQ ID NO: 45899 - protein, 9 aa, synthetic construct
GGGGLDTVA

SEQ ID NO: 45900 - protein, 9 aa, synthetic construct
GGGGKDQLD

SEQ ID NO: 45901 - protein, 9 aa, synthetic construct
GGGGKDNLS

SEQ ID NO: 45902 - protein, 9 aa, synthetic construct
GGGGKDMLS

SEQ ID NO: 45903 - protein, 9 aa, synthetic construct
GGGGKDMFV

SEQ ID NO: 45904 - protein, 9 aa, synthetic construct
GGGGIDHFR

SEQ ID NO: 45905 - protein, 9 aa, synthetic construct
GGGGIDIAL

SEQ ID NO: 45906 - protein, 9 aa, synthetic construct
GGGGIDIIV

SEQ ID NO: 45907 - protein, 9 aa, synthetic construct
GGGGIDILF

SEQ ID NO: 45908 - protein, 9 aa, synthetic construct
GGGGIDILR

SEQ ID NO: 45909 - protein, 9 aa, synthetic construct
GGGGIDILY

SEQ ID NO: 45910 - protein, 9 aa, synthetic construct
GGGGIDIVF

SEQ ID NO: 45911 - protein, 9 aa, synthetic construct
GGGGIDKLY

SEQ ID NO: 45912 - protein, 9 aa, synthetic construct
GGGGIDLAS

SEQ ID NO: 45913 - protein, 9 aa, synthetic construct
GGGGIDLAT

SEQ ID NO: 45914 - protein, 9 aa, synthetic construct
GGGGIDLFM

SEQ ID NO: 45915 - protein, 9 aa, synthetic construct
GGGGIDLIV

SEQ ID NO: 45916 - protein, 9 aa, synthetic construct
GGGGIDLLA

SEQ ID NO: 45917 - protein, 9 aa, synthetic construct
GGGGIDLLH

SEQ ID NO: 45918 - protein, 9 aa, synthetic construct
GGGGIDLLK

SEQ ID NO: 45919 - protein, 9 aa, synthetic construct
GGGGIDLLS

SEQ ID NO: 45920 - protein, 9 aa, synthetic construct
GGGGIDLLY

SEQ ID NO: 45921 - protein, 9 aa, synthetic construct
GGGGIDLVD

SEQ ID NO: 45922 - protein, 9 aa, synthetic construct
GGGGIDNLF

SEQ ID NO: 45923 - protein, 9 aa, synthetic construct
GGGGIDQAD

SEQ ID NO: 45924 - protein, 9 aa, synthetic construct
GGGGIDQLD

SEQ ID NO: 45925 - protein, 9 aa, synthetic construct
GGGGIDQLF

SEQ ID NO: 45926 - protein, 9 aa, synthetic construct
GGGGIDRAV

SEQ ID NO: 45927 - protein, 9 aa, synthetic construct
GGGGIDRFI

SEQ ID NO: 45928 - protein, 9 aa, synthetic construct
GGGGIDRLI

SEQ ID NO: 45929 - protein, 9 aa, synthetic construct
GGGGIDRVS

SEQ ID NO: 45930 - protein, 9 aa, synthetic construct
GGGGIDSAA

SEQ ID NO: 45931 - protein, 9 aa, synthetic construct
GGGGIDSLE

SEQ ID NO: 45932 - protein, 9 aa, synthetic construct
GGGGIDSLF

SEQ ID NO: 45933 - protein, 9 aa, synthetic construct
GGGGIDGFN

SEQ ID NO: 45934 - protein, 9 aa, synthetic construct
GGGGIDFVS

SEQ ID NO: 45935 - protein, 9 aa, synthetic construct
GGGGIDFVN

SEQ ID NO: 45936 - protein, 9 aa, synthetic construct
GGGGHDVLR

SEQ ID NO: 45937 - protein, 9 aa, synthetic construct
GGGGHDTVR

SEQ ID NO: 45938 - protein, 9 aa, synthetic construct
GGGGHDTVV

SEQ ID NO: 45939 - protein, 9 aa, synthetic construct
GGGGHDTVY

SEQ ID NO: 45940 - protein, 9 aa, synthetic construct
GGGGHDVAT

SEQ ID NO: 45941 - protein, 9 aa, synthetic construct
GGGGHDVFG

SEQ ID NO: 45942 - protein, 9 aa, synthetic construct
GGGGHDVFK

SEQ ID NO: 45943 - protein, 9 aa, synthetic construct
GGGGHDVFY

SEQ ID NO: 45944 - protein, 9 aa, synthetic construct
GGGGHDVIA

SEQ ID NO: 45945 - protein, 9 aa, synthetic construct
GGGGHDVIH

SEQ ID NO: 45946 - protein, 9 aa, synthetic construct
GGGGHDVLA

SEQ ID NO: 45947 - protein, 9 aa, synthetic construct
GGGGHDVLG

SEQ ID NO: 45948 - protein, 9 aa, synthetic construct
GGGGHDVLH

SEQ ID NO: 45949 - protein, 9 aa, synthetic construct
GGGGHDVLN

SEQ ID NO: 45950 - protein, 9 aa, synthetic construct
GGGGHDVVE

SEQ ID NO: 45951 - protein, 9 aa, synthetic construct
GGGGIDFMQ

SEQ ID NO: 45952 - protein, 9 aa, synthetic construct
GGGGHDVVS

SEQ ID NO: 45953 - protein, 9 aa, synthetic construct
GGGGHDWIA

SEQ ID NO: 45954 - protein, 9 aa, synthetic construct
GGGGHDWLL

SEQ ID NO: 45955 - protein, 9 aa, synthetic construct
GGGGHDYLR

SEQ ID NO: 45956 - protein, 9 aa, synthetic construct
GGGGIDAAS

SEQ ID NO: 45957 - protein, 9 aa, synthetic construct
GGGGIDAFH

SEQ ID NO: 45958 - protein, 9 aa, synthetic construct
GGGGIDAFR

SEQ ID NO: 45959 - protein, 9 aa, synthetic construct
GGGGIDALF

SEQ ID NO: 45960 - protein, 9 aa, synthetic construct
GGGGIDAMT

SEQ ID NO: 45961 - protein, 9 aa, synthetic construct
GGGGIDDLY

SEQ ID NO: 45962 - protein, 9 aa, synthetic construct
GGGGIDEMT

SEQ ID NO: 45963 - protein, 9 aa, synthetic construct
GGGGIDFLD

SEQ ID NO: 45964 - protein, 9 aa, synthetic construct
GGGGIDFLT

SEQ ID NO: 45965 - protein, 9 aa, synthetic construct
GGGGIDSLN

SEQ ID NO: 45966 - protein, 9 aa, synthetic construct
GGGGIDSLS

SEQ ID NO: 45967 - protein, 9 aa, synthetic construct
GGGGIDSMS

SEQ ID NO: 45968 - protein, 9 aa, synthetic construct
GGGGKDILY

SEQ ID NO: 45969 - protein, 9 aa, synthetic construct
GGGGKDDLY

SEQ ID NO: 45970 - protein, 9 aa, synthetic construct
GGGGKDEFV

SEQ ID NO: 45971 - protein, 9 aa, synthetic construct
GGGGKDEIE

SEQ ID NO: 45972 - protein, 9 aa, synthetic construct
GGGGKDEIF

SEQ ID NO: 45973 - protein, 9 aa, synthetic construct
GGGGKDFFA

SEQ ID NO: 45974 - protein, 9 aa, synthetic construct
GGGGKDFLS

SEQ ID NO: 45975 - protein, 9 aa, synthetic construct
GGGGKDFLY

SEQ ID NO: 45976 - protein, 9 aa, synthetic construct
GGGGKDHLD

SEQ ID NO: 45977 - protein, 9 aa, synthetic construct
GGGGKDHLY

SEQ ID NO: 45978 - protein, 9 aa, synthetic construct
GGGGKDIFQ

SEQ ID NO: 45979 - protein, 9 aa, synthetic construct
GGGGKDIFT

SEQ ID NO: 45980 - protein, 9 aa, synthetic construct
GGGGKDILE

SEQ ID NO: 45981 - protein, 9 aa, synthetic construct
GGGGKDILK

SEQ ID NO: 45982 - protein, 9 aa, synthetic construct
GGGGKDIVW

SEQ ID NO: 45983 - protein, 9 aa, synthetic construct
GGGGKDALW

SEQ ID NO: 45984 - protein, 9 aa, synthetic construct
GGGGKDKIG

SEQ ID NO: 45985 - protein, 9 aa, synthetic construct
GGGGKDKLF

SEQ ID NO: 45986 - protein, 9 aa, synthetic construct
GGGGKDKLN

SEQ ID NO: 45987 - protein, 9 aa, synthetic construct
GGGGKDKLT

SEQ ID NO: 45988 - protein, 9 aa, synthetic construct
GGGGKDKLV

SEQ ID NO: 45989 - protein, 9 aa, synthetic construct
GGGGKDLLA

SEQ ID NO: 45990 - protein, 9 aa, synthetic construct
GGGGKDLLE

SEQ ID NO: 45991 - protein, 9 aa, synthetic construct
GGGGKDLLK

SEQ ID NO: 45992 - protein, 9 aa, synthetic construct
GGGGKDLLN

SEQ ID NO: 45993 - protein, 9 aa, synthetic construct
GGGGKDLLR

SEQ ID NO: 45994 - protein, 9 aa, synthetic construct
GGGGKDLLT

SEQ ID NO: 45995 - protein, 9 aa, synthetic construct
GGGGKDLLV

SEQ ID NO: 45996 - protein, 9 aa, synthetic construct
GGGGKDLVK

SEQ ID NO: 45997 - protein, 9 aa, synthetic construct
GGGGKDDLE

SEQ ID NO: 45998 - protein, 9 aa, synthetic construct
GGGGKDALN

SEQ ID NO: 45999 - protein, 9 aa, synthetic construct
GGGGIDTAF

SEQ ID NO: 46000 - protein, 9 aa, synthetic construct
GGGGIDVIR

SEQ ID NO: 46001 - protein, 9 aa, synthetic construct
GGGGIDTAT

SEQ ID NO: 46002 - protein, 9 aa, synthetic construct
GGGGIDTFA

SEQ ID NO: 46003 - protein, 9 aa, synthetic construct
GGGGIDTFH

SEQ ID NO: 46004 - protein, 9 aa, synthetic construct
GGGGIDTFR

SEQ ID NO: 46005 - protein, 9 aa, synthetic construct
GGGGIDTIE

SEQ ID NO: 46006 - protein, 9 aa, synthetic construct
GGGGIDTIF

SEQ ID NO: 46007 - protein, 9 aa, synthetic construct
GGGGIDTIN

SEQ ID NO: 46008 - protein, 9 aa, synthetic construct
GGGGIDTIS

SEQ ID NO: 46009 - protein, 9 aa, synthetic construct
GGGGIDTMD

SEQ ID NO: 46010 - protein, 9 aa, synthetic construct
GGGGIDTVY

SEQ ID NO: 46011 - protein, 9 aa, synthetic construct
GGGGIDVFV

SEQ ID NO: 46012 - protein, 9 aa, synthetic construct
GGGGIDVID

SEQ ID NO: 46013 - protein, 9 aa, synthetic construct
GGGGIDVIN

SEQ ID NO: 46014 - protein, 9 aa, synthetic construct
GGGGIDVIT

SEQ ID NO: 46015 - protein, 9 aa, synthetic construct
GGGGKDAIS

SEQ ID NO: 46016 - protein, 9 aa, synthetic construct
GGGGIDVLD

SEQ ID NO: 46017 - protein, 9 aa, synthetic construct
GGGGIDVLF

SEQ ID NO: 46018 - protein, 9 aa, synthetic construct
GGGGIDVLI

SEQ ID NO: 46019 - protein, 9 aa, synthetic construct
GGGGIDVLR

SEQ ID NO: 46020 - protein, 9 aa, synthetic construct
GGGGIDVLS

SEQ ID NO: 46021 - protein, 9 aa, synthetic construct
GGGGIDVMV

SEQ ID NO: 46022 - protein, 9 aa, synthetic construct
GGGGIDWLD

SEQ ID NO: 46023 - protein, 9 aa, synthetic construct
GGGGIDWLY

SEQ ID NO: 46024 - protein, 9 aa, synthetic construct
GGGGIDYAW

SEQ ID NO: 46025 - protein, 9 aa, synthetic construct
GGGGIDYFI

SEQ ID NO: 46026 - protein, 9 aa, synthetic construct
GGGGIDYMY

SEQ ID NO: 46027 - protein, 9 aa, synthetic construct
GGGGIDYVS

SEQ ID NO: 46028 - protein, 9 aa, synthetic construct
GGGGKDAAS

SEQ ID NO: 46029 - protein, 9 aa, synthetic construct
GGGGEDSLY

SEQ ID NO: 46030 - protein, 9 aa, synthetic construct
GGGGEDSLS

SEQ ID NO: 46031 - protein, 9 aa, synthetic construct
GGGGEDSLF

SEQ ID NO: 46032 - protein, 9 aa, synthetic construct
GGGGADRVY

SEQ ID NO: 46033 - protein, 9 aa, synthetic construct
GGGGADNMD

SEQ ID NO: 46034 - protein, 9 aa, synthetic construct
GGGGADNMI

SEQ ID NO: 46035 - protein, 9 aa, synthetic construct
GGGGADNMS

SEQ ID NO: 46036 - protein, 9 aa, synthetic construct
GGGGADNVF

SEQ ID NO: 46037 - protein, 9 aa, synthetic construct
GGGGADNVQ

SEQ ID NO: 46038 - protein, 9 aa, synthetic construct
GGGGADQIF

SEQ ID NO: 46039 - protein, 9 aa, synthetic construct
GGGGADQIN

SEQ ID NO: 46040 - protein, 9 aa, synthetic construct
GGGGADQLG

SEQ ID NO: 46041 - protein, 9 aa, synthetic construct
GGGGADQLL

SEQ ID NO: 46042 - protein, 9 aa, synthetic construct
GGGGADQMA

SEQ ID NO: 46043 - protein, 9 aa, synthetic construct
GGGGADQVN

SEQ ID NO: 46044 - protein, 9 aa, synthetic construct
GGGGADQVY

SEQ ID NO: 46045 - protein, 9 aa, synthetic construct
GGGGADQYL

SEQ ID NO: 46046 - protein, 9 aa, synthetic construct
GGGGADQYY

SEQ ID NO: 46047 - protein, 9 aa, synthetic construct
GGGGADRAD

SEQ ID NO: 46048 - protein, 9 aa, synthetic construct
GGGGADRFD

SEQ ID NO: 46049 - protein, 9 aa, synthetic construct
GGGGADRFY

SEQ ID NO: 46050 - protein, 9 aa, synthetic construct
GGGGADRIA

SEQ ID NO: 46051 - protein, 9 aa, synthetic construct
GGGGADRIH

SEQ ID NO: 46052 - protein, 9 aa, synthetic construct
GGGGADRII

SEQ ID NO: 46053 - protein, 9 aa, synthetic construct
GGGGADRIK

SEQ ID NO: 46054 - protein, 9 aa, synthetic construct
GGGGADRIR

SEQ ID NO: 46055 - protein, 9 aa, synthetic construct
GGGGADRLK

SEQ ID NO: 46056 - protein, 9 aa, synthetic construct
GGGGADRLM

SEQ ID NO: 46057 - protein, 9 aa, synthetic construct
GGGGADRMI

SEQ ID NO: 46058 - protein, 9 aa, synthetic construct
GGGGADRML

SEQ ID NO: 46059 - protein, 9 aa, synthetic construct
GGGGADRMV

SEQ ID NO: 46060 - protein, 9 aa, synthetic construct
GGGGADRVA

SEQ ID NO: 46061 - protein, 9 aa, synthetic construct
GGGGADRVF

SEQ ID NO: 46062 - protein, 9 aa, synthetic construct
GGGGADNLY

SEQ ID NO: 46063 - protein, 9 aa, synthetic construct
GGGGADNLQ

SEQ ID NO: 46064 - protein, 9 aa, synthetic construct
GGGGADNLL

SEQ ID NO: 46065 - protein, 9 aa, synthetic construct
GGGGADLVL

SEQ ID NO: 46066 - protein, 9 aa, synthetic construct
GGGGADLFY

SEQ ID NO: 46067 - protein, 9 aa, synthetic construct
GGGGADLIN

SEQ ID NO: 46068 - protein, 9 aa, synthetic construct
GGGGADLIS

SEQ ID NO: 46069 - protein, 9 aa, synthetic construct
GGGGADLLC

SEQ ID NO: 46070 - protein, 9 aa, synthetic construct
GGGGADLLL

SEQ ID NO: 46071 - protein, 9 aa, synthetic construct
GGGGADLLM

SEQ ID NO: 46072 - protein, 9 aa, synthetic construct
GGGGADLLQ

SEQ ID NO: 46073 - protein, 9 aa, synthetic construct
GGGGADLLW

SEQ ID NO: 46074 - protein, 9 aa, synthetic construct
GGGGADLML

SEQ ID NO: 46075 - protein, 9 aa, synthetic construct
GGGGADLMY

SEQ ID NO: 46076 - protein, 9 aa, synthetic construct
GGGGADLVA

SEQ ID NO: 46077 - protein, 9 aa, synthetic construct
GGGGADLVD

SEQ ID NO: 46078 - protein, 9 aa, synthetic construct
GGGGADLVK

SEQ ID NO: 46079 - protein, 9 aa, synthetic construct
GGGGADLVQ

SEQ ID NO: 46080 - protein, 9 aa, synthetic construct
GGGGADNIA

SEQ ID NO: 46081 - protein, 9 aa, synthetic construct
GGGGADLVR

SEQ ID NO: 46082 - protein, 9 aa, synthetic construct
GGGGADLYV

SEQ ID NO: 46083 - protein, 9 aa, synthetic construct
GGGGADMFL

SEQ ID NO: 46084 - protein, 9 aa, synthetic construct
GGGGADMID

SEQ ID NO: 46085 - protein, 9 aa, synthetic construct
GGGGADMIH

SEQ ID NO: 46086 - protein, 9 aa, synthetic construct
GGGGADMIY

SEQ ID NO: 46087 - protein, 9 aa, synthetic construct
GGGGADMLA

SEQ ID NO: 46088 - protein, 9 aa, synthetic construct
GGGGADMLH

SEQ ID NO: 46089 - protein, 9 aa, synthetic construct
GGGGADMLI

SEQ ID NO: 46090 - protein, 9 aa, synthetic construct
GGGGADMLK

SEQ ID NO: 46091 - protein, 9 aa, synthetic construct
GGGGADMLY

SEQ ID NO: 46092 - protein, 9 aa, synthetic construct
GGGGADMVR

SEQ ID NO: 46093 - protein, 9 aa, synthetic construct
GGGGADNFK

SEQ ID NO: 46094 - protein, 9 aa, synthetic construct
GGGGADRVL

SEQ ID NO: 46095 - protein, 9 aa, synthetic construct
GGGGADSAT

SEQ ID NO: 46096 - protein, 9 aa, synthetic construct
GGGGEDSIE

SEQ ID NO: 46097 - protein, 9 aa, synthetic construct
GGGGADSFD

SEQ ID NO: 46098 - protein, 9 aa, synthetic construct
GGGGADVLH

SEQ ID NO: 46099 - protein, 9 aa, synthetic construct
GGGGADVMA

SEQ ID NO: 46100 - protein, 9 aa, synthetic construct
GGGGADVMH

SEQ ID NO: 46101 - protein, 9 aa, synthetic construct
GGGGADVMN

SEQ ID NO: 46102 - protein, 9 aa, synthetic construct
GGGGADVMV

SEQ ID NO: 46103 - protein, 9 aa, synthetic construct
GGGGADVVA

SEQ ID NO: 46104 - protein, 9 aa, synthetic construct
GGGGADVVD

SEQ ID NO: 46105 - protein, 9 aa, synthetic construct
GGGGADVYQ

SEQ ID NO: 46106 - protein, 9 aa, synthetic construct
GGGGADWFR

SEQ ID NO: 46107 - protein, 9 aa, synthetic construct
GGGGADWII

SEQ ID NO: 46108 - protein, 9 aa, synthetic construct
GGGGADWLA

SEQ ID NO: 46109 - protein, 9 aa, synthetic construct
GGGGADWLE

SEQ ID NO: 46110 - protein, 9 aa, synthetic construct
GGGGADWLF

SEQ ID NO: 46111 - protein, 9 aa, synthetic construct
GGGGADYID

SEQ ID NO: 46112 - protein, 9 aa, synthetic construct
GGGGADYIL

SEQ ID NO: 46113 - protein, 9 aa, synthetic construct
GGGGADYIQ

SEQ ID NO: 46114 - protein, 9 aa, synthetic construct
GGGGADYLA

SEQ ID NO: 46115 - protein, 9 aa, synthetic construct
GGGGADYLE

SEQ ID NO: 46116 - protein, 9 aa, synthetic construct
GGGGADYLS

SEQ ID NO: 46117 - protein, 9 aa, synthetic construct
GGGGADYLT

SEQ ID NO: 46118 - protein, 9 aa, synthetic construct
GGGGADYLV

SEQ ID NO: 46119 - protein, 9 aa, synthetic construct
GGGGADYLY

SEQ ID NO: 46120 - protein, 9 aa, synthetic construct
GGGGADYMD

SEQ ID NO: 46121 - protein, 9 aa, synthetic construct
GGGGADYVS

SEQ ID NO: 46122 - protein, 9 aa, synthetic construct
GGGGCDTLY

SEQ ID NO: 46123 - protein, 9 aa, synthetic construct
GGGGCDVLR

SEQ ID NO: 46124 - protein, 9 aa, synthetic construct
GGGGDDAID

SEQ ID NO: 46125 - protein, 9 aa, synthetic construct
GGGGDDAIE

SEQ ID NO: 46126 - protein, 9 aa, synthetic construct
GGGGDDAIF

SEQ ID NO: 46127 - protein, 9 aa, synthetic construct
GGGGADVII

SEQ ID NO: 46128 - protein, 9 aa, synthetic construct
GGGGADVIG

SEQ ID NO: 46129 - protein, 9 aa, synthetic construct
GGGGADVFM

SEQ ID NO: 46130 - protein, 9 aa, synthetic construct
GGGGADTMH

SEQ ID NO: 46131 - protein, 9 aa, synthetic construct
GGGGADSLG

SEQ ID NO: 46132 - protein, 9 aa, synthetic construct
GGGGADSLK

SEQ ID NO: 46133 - protein, 9 aa, synthetic construct
GGGGADSMD

SEQ ID NO: 46134 - protein, 9 aa, synthetic construct
GGGGADSME

SEQ ID NO: 46135 - protein, 9 aa, synthetic construct
GGGGADSYV

SEQ ID NO: 46136 - protein, 9 aa, synthetic construct
GGGGADTAV

SEQ ID NO: 46137 - protein, 9 aa, synthetic construct
GGGGADTFK

SEQ ID NO: 46138 - protein, 9 aa, synthetic construct
GGGGADTFQ

SEQ ID NO: 46139 - protein, 9 aa, synthetic construct
GGGGADTIV

SEQ ID NO: 46140 - protein, 9 aa, synthetic construct
GGGGADTIW

SEQ ID NO: 46141 - protein, 9 aa, synthetic construct
GGGGADTMC

SEQ ID NO: 46142 - protein, 9 aa, synthetic construct
GGGGADTMF

SEQ ID NO: 46143 - protein, 9 aa, synthetic construct
GGGGADTMG

SEQ ID NO: 46144 - protein, 9 aa, synthetic construct
GGGGADTMR

SEQ ID NO: 46145 - protein, 9 aa, synthetic construct
GGGGADVFE

SEQ ID NO: 46146 - protein, 9 aa, synthetic construct
GGGGADTMY

SEQ ID NO: 46147 - protein, 9 aa, synthetic construct
GGGGADTVA

SEQ ID NO: 46148 - protein, 9 aa, synthetic construct
GGGGADTVE

SEQ ID NO: 46149 - protein, 9 aa, synthetic construct
GGGGADTVF

SEQ ID NO: 46150 - protein, 9 aa, synthetic construct
GGGGADTVI

SEQ ID NO: 46151 - protein, 9 aa, synthetic construct
GGGGADTVN

SEQ ID NO: 46152 - protein, 9 aa, synthetic construct
GGGGADTVQ

SEQ ID NO: 46153 - protein, 9 aa, synthetic construct
GGGGADTVR

SEQ ID NO: 46154 - protein, 9 aa, synthetic construct
GGGGADTVW

SEQ ID NO: 46155 - protein, 9 aa, synthetic construct
GGGGADTYA

SEQ ID NO: 46156 - protein, 9 aa, synthetic construct
GGGGADTYS

SEQ ID NO: 46157 - protein, 9 aa, synthetic construct
GGGGADTYY

SEQ ID NO: 46158 - protein, 9 aa, synthetic construct
GGGGADVFD

SEQ ID NO: 46159 - protein, 9 aa, synthetic construct
GGGGADLFQ

SEQ ID NO: 46160 - protein, 9 aa, synthetic construct
GGGGADLFL

SEQ ID NO: 46161 - protein, 9 aa, synthetic construct
GGGGADLFH

SEQ ID NO: 46162 - protein, 9 aa, synthetic construct
GGGGADLFD

SEQ ID NO: 46163 - protein, 9 aa, synthetic construct
GGFGYDVLI

SEQ ID NO: 46164 - protein, 9 aa, synthetic construct
GGFGYDVVH

SEQ ID NO: 46165 - protein, 9 aa, synthetic construct
GGFGYDYLR

SEQ ID NO: 46166 - protein, 9 aa, synthetic construct
GGGGADAFN

SEQ ID NO: 46167 - protein, 9 aa, synthetic construct
GGGGADAFW

SEQ ID NO: 46168 - protein, 9 aa, synthetic construct
GGGGADAIA

SEQ ID NO: 46169 - protein, 9 aa, synthetic construct
GGGGADAIE

SEQ ID NO: 46170 - protein, 9 aa, synthetic construct
GGGGADAIY

SEQ ID NO: 46171 - protein, 9 aa, synthetic construct
GGGGADALE

SEQ ID NO: 46172 - protein, 9 aa, synthetic construct
GGGGADALH

SEQ ID NO: 46173 - protein, 9 aa, synthetic construct
GGGGADAMD

SEQ ID NO: 46174 - protein, 9 aa, synthetic construct
GGGGADAVD

SEQ ID NO: 46175 - protein, 9 aa, synthetic construct
GGGGADAVL

SEQ ID NO: 46176 - protein, 9 aa, synthetic construct
GGGGADDFD

SEQ ID NO: 46177 - protein, 9 aa, synthetic construct
GGGGADDFI

SEQ ID NO: 46178 - protein, 9 aa, synthetic construct
GGGGADDFN

SEQ ID NO: 46179 - protein, 9 aa, synthetic construct
GGGGADDIH

SEQ ID NO: 46180 - protein, 9 aa, synthetic construct
GGGGADDIN

SEQ ID NO: 46181 - protein, 9 aa, synthetic construct
GGGGADDIR

SEQ ID NO: 46182 - protein, 9 aa, synthetic construct
GGGGADDIS

SEQ ID NO: 46183 - protein, 9 aa, synthetic construct
GGGGADDIT

SEQ ID NO: 46184 - protein, 9 aa, synthetic construct
GGGGADDIY

SEQ ID NO: 46185 - protein, 9 aa, synthetic construct
GGGGADDLF

SEQ ID NO: 46186 - protein, 9 aa, synthetic construct
GGGGADDLI

SEQ ID NO: 46187 - protein, 9 aa, synthetic construct
GGGGADDLY

SEQ ID NO: 46188 - protein, 9 aa, synthetic construct
GGGGADDMD

SEQ ID NO: 46189 - protein, 9 aa, synthetic construct
GGGGADDMR

SEQ ID NO: 46190 - protein, 9 aa, synthetic construct
GGGGADDMT

SEQ ID NO: 46191 - protein, 9 aa, synthetic construct
GGGGADEFH

SEQ ID NO: 46192 - protein, 9 aa, synthetic construct
GGFGYDTLT

SEQ ID NO: 46193 - protein, 9 aa, synthetic construct
GGFGYDTLE

SEQ ID NO: 46194 - protein, 9 aa, synthetic construct
GGFGYDRLQ

SEQ ID NO: 46195 - protein, 9 aa, synthetic construct
GGFGVDTMD

SEQ ID NO: 46196 - protein, 9 aa, synthetic construct
GGFGVDLIL

SEQ ID NO: 46197 - protein, 9 aa, synthetic construct
GGFGVDLLN

SEQ ID NO: 46198 - protein, 9 aa, synthetic construct
GGFGVDLVI

SEQ ID NO: 46199 - protein, 9 aa, synthetic construct
GGFGVDNII

SEQ ID NO: 46200 - protein, 9 aa, synthetic construct
GGFGVDQLI

SEQ ID NO: 46201 - protein, 9 aa, synthetic construct
GGFGVDQVI

SEQ ID NO: 46202 - protein, 9 aa, synthetic construct
GGFGVDRLI

SEQ ID NO: 46203 - protein, 9 aa, synthetic construct
GGFGVDRLY

SEQ ID NO: 46204 - protein, 9 aa, synthetic construct
GGFGVDSIT

SEQ ID NO: 46205 - protein, 9 aa, synthetic construct
GGFGVDSLF

SEQ ID NO: 46206 - protein, 9 aa, synthetic construct
GGFGVDTID

SEQ ID NO: 46207 - protein, 9 aa, synthetic construct
GGFGVDTLN

SEQ ID NO: 46208 - protein, 9 aa, synthetic construct
GGFGVDTLY

SEQ ID NO: 46209 - protein, 9 aa, synthetic construct
GGFGVDTMT

SEQ ID NO: 46210 - protein, 9 aa, synthetic construct
GGFGYDRAN

SEQ ID NO: 46211 - protein, 9 aa, synthetic construct
GGFGVDTVM

SEQ ID NO: 46212 - protein, 9 aa, synthetic construct
GGFGVDTVR

SEQ ID NO: 46213 - protein, 9 aa, synthetic construct
GGFGVDVAI

SEQ ID NO: 46214 - protein, 9 aa, synthetic construct
GGFGWDILR

SEQ ID NO: 46215 - protein, 9 aa, synthetic construct
GGFGWDRLI

SEQ ID NO: 46216 - protein, 9 aa, synthetic construct
GGFGWDVAS

SEQ ID NO: 46217 - protein, 9 aa, synthetic construct
GGFGYDEIY

SEQ ID NO: 46218 - protein, 9 aa, synthetic construct
GGFGYDELQ

SEQ ID NO: 46219 - protein, 9 aa, synthetic construct
GGFGYDEMR

SEQ ID NO: 46220 - protein, 9 aa, synthetic construct
GGFGYDKMI

SEQ ID NO: 46221 - protein, 9 aa, synthetic construct
GGFGYDLMN

SEQ ID NO: 46222 - protein, 9 aa, synthetic construct
GGFGYDQAN

SEQ ID NO: 46223 - protein, 9 aa, synthetic construct
GGFGYDQMR

SEQ ID NO: 46224 - protein, 9 aa, synthetic construct
GGGGADEIA

SEQ ID NO: 46225 - protein, 9 aa, synthetic construct
GGGGADEID

SEQ ID NO: 46226 - protein, 9 aa, synthetic construct
GGGGADEII

SEQ ID NO: 46227 - protein, 9 aa, synthetic construct
GGGGADIMS

SEQ ID NO: 46228 - protein, 9 aa, synthetic construct
GGGGADIFA

SEQ ID NO: 46229 - protein, 9 aa, synthetic construct
GGGGADIFG

SEQ ID NO: 46230 - protein, 9 aa, synthetic construct
GGGGADIFH

SEQ ID NO: 46231 - protein, 9 aa, synthetic construct
GGGGADIFQ

SEQ ID NO: 46232 - protein, 9 aa, synthetic construct
GGGGADIFY

SEQ ID NO: 46233 - protein, 9 aa, synthetic construct
GGGGADIIN

SEQ ID NO: 46234 - protein, 9 aa, synthetic construct
GGGGADIIS

SEQ ID NO: 46235 - protein, 9 aa, synthetic construct
GGGGADIIV

SEQ ID NO: 46236 - protein, 9 aa, synthetic construct
GGGGADILQ

SEQ ID NO: 46237 - protein, 9 aa, synthetic construct
GGGGADILW

SEQ ID NO: 46238 - protein, 9 aa, synthetic construct
GGGGADIMA

SEQ ID NO: 46239 - protein, 9 aa, synthetic construct
GGGGADIMD

SEQ ID NO: 46240 - protein, 9 aa, synthetic construct
GGGGADIMR

SEQ ID NO: 46241 - protein, 9 aa, synthetic construct
GGGGADIMY

SEQ ID NO: 46242 - protein, 9 aa, synthetic construct
GGGGADIAI

SEQ ID NO: 46243 - protein, 9 aa, synthetic construct
GGGGADIVA

SEQ ID NO: 46244 - protein, 9 aa, synthetic construct
GGGGADIVN

SEQ ID NO: 46245 - protein, 9 aa, synthetic construct
GGGGADIYF

SEQ ID NO: 46246 - protein, 9 aa, synthetic construct
GGGGADIYY

SEQ ID NO: 46247 - protein, 9 aa, synthetic construct
GGGGADKFL

SEQ ID NO: 46248 - protein, 9 aa, synthetic construct
GGGGADKID

SEQ ID NO: 46249 - protein, 9 aa, synthetic construct
GGGGADKIS

SEQ ID NO: 46250 - protein, 9 aa, synthetic construct
GGGGADKLA

SEQ ID NO: 46251 - protein, 9 aa, synthetic construct
GGGGADKLG

SEQ ID NO: 46252 - protein, 9 aa, synthetic construct
GGGGADKLK

SEQ ID NO: 46253 - protein, 9 aa, synthetic construct
GGGGADKML

SEQ ID NO: 46254 - protein, 9 aa, synthetic construct
GGGGADKMY

SEQ ID NO: 46255 - protein, 9 aa, synthetic construct
GGGGADLFA

SEQ ID NO: 46256 - protein, 9 aa, synthetic construct
GGGGADIAV

SEQ ID NO: 46257 - protein, 9 aa, synthetic construct
GGGGADHVH

SEQ ID NO: 46258 - protein, 9 aa, synthetic construct
GGGGADEIT

SEQ ID NO: 46259 - protein, 9 aa, synthetic construct
GGGGADFLN

SEQ ID NO: 46260 - protein, 9 aa, synthetic construct
GGGGADEIY

SEQ ID NO: 46261 - protein, 9 aa, synthetic construct
GGGGADELA

SEQ ID NO: 46262 - protein, 9 aa, synthetic construct
GGGGADELH

SEQ ID NO: 46263 - protein, 9 aa, synthetic construct
GGGGADELT

SEQ ID NO: 46264 - protein, 9 aa, synthetic construct
GGGGADEMA

SEQ ID NO: 46265 - protein, 9 aa, synthetic construct
GGGGADEMH

SEQ ID NO: 46266 - protein, 9 aa, synthetic construct
GGGGADEYR

SEQ ID NO: 46267 - protein, 9 aa, synthetic construct
GGGGADFAF

SEQ ID NO: 46268 - protein, 9 aa, synthetic construct
GGGGADFFD

SEQ ID NO: 46269 - protein, 9 aa, synthetic construct
GGGGADFIA

SEQ ID NO: 46270 - protein, 9 aa, synthetic construct
GGGGADFIS

SEQ ID NO: 46271 - protein, 9 aa, synthetic construct
GGGGADFLG

SEQ ID NO: 46272 - protein, 9 aa, synthetic construct
GGGGADFLM

SEQ ID NO: 46273 - protein, 9 aa, synthetic construct
GGGGADFLR

SEQ ID NO: 46274 - protein, 9 aa, synthetic construct
GGGGADHVE

SEQ ID NO: 46275 - protein, 9 aa, synthetic construct
GGGGADFLY

SEQ ID NO: 46276 - protein, 9 aa, synthetic construct
GGGGADGIA

SEQ ID NO: 46277 - protein, 9 aa, synthetic construct
GGGGADGID

SEQ ID NO: 46278 - protein, 9 aa, synthetic construct
GGGGADGIT

SEQ ID NO: 46279 - protein, 9 aa, synthetic construct
GGGGADGIW

SEQ ID NO: 46280 - protein, 9 aa, synthetic construct
GGGGADGLF

SEQ ID NO: 46281 - protein, 9 aa, synthetic construct
GGGGADGLR

SEQ ID NO: 46282 - protein, 9 aa, synthetic construct
GGGGADGLS

SEQ ID NO: 46283 - protein, 9 aa, synthetic construct
GGGGADHFQ

SEQ ID NO: 46284 - protein, 9 aa, synthetic construct
GGGGADHFR

SEQ ID NO: 46285 - protein, 9 aa, synthetic construct
GGGGADHIF

SEQ ID NO: 46286 - protein, 9 aa, synthetic construct
GGGGADHLE

SEQ ID NO: 46287 - protein, 9 aa, synthetic construct
GGGGADHLF

SEQ ID NO: 46288 - protein, 9 aa, synthetic construct
GGGGDDAIN

SEQ ID NO: 46289 - protein, 9 aa, synthetic construct
GGGGDDAIV

SEQ ID NO: 46290 - protein, 9 aa, synthetic construct
GGGGDDALA

SEQ ID NO: 46291 - protein, 9 aa, synthetic construct
GGGGDDQLL

SEQ ID NO: 46292 - protein, 9 aa, synthetic construct
GGGGDDSML

SEQ ID NO: 46293 - protein, 9 aa, synthetic construct
GGGGDDSMS

SEQ ID NO: 46294 - protein, 9 aa, synthetic construct
GGGGDDSVA

SEQ ID NO: 46295 - protein, 9 aa, synthetic construct
GGGGDDSVE

SEQ ID NO: 46296 - protein, 9 aa, synthetic construct
GGGGDDSVL

SEQ ID NO: 46297 - protein, 9 aa, synthetic construct
GGGGDDSVT

SEQ ID NO: 46298 - protein, 9 aa, synthetic construct
GGGGDDSYR

SEQ ID NO: 46299 - protein, 9 aa, synthetic construct
GGGGDDTAV

SEQ ID NO: 46300 - protein, 9 aa, synthetic construct
GGGGDDTFF

SEQ ID NO: 46301 - protein, 9 aa, synthetic construct
GGGGDDTFG

SEQ ID NO: 46302 - protein, 9 aa, synthetic construct
GGGGDDTFI

SEQ ID NO: 46303 - protein, 9 aa, synthetic construct
GGGGDDTFL

SEQ ID NO: 46304 - protein, 9 aa, synthetic construct
GGGGDDTFN

SEQ ID NO: 46305 - protein, 9 aa, synthetic construct
GGGGDDTFT

SEQ ID NO: 46306 - protein, 9 aa, synthetic construct
GGGGDDTIK

SEQ ID NO: 46307 - protein, 9 aa, synthetic construct
GGGGDDTIS

SEQ ID NO: 46308 - protein, 9 aa, synthetic construct
GGGGDDTIW

SEQ ID NO: 46309 - protein, 9 aa, synthetic construct
GGGGDDTMD

SEQ ID NO: 46310 - protein, 9 aa, synthetic construct
GGGGDDTME

SEQ ID NO: 46311 - protein, 9 aa, synthetic construct
GGGGDDTMI

SEQ ID NO: 46312 - protein, 9 aa, synthetic construct
GGGGDDTMY

SEQ ID NO: 46313 - protein, 9 aa, synthetic construct
GGGGDDTVF

SEQ ID NO: 46314 - protein, 9 aa, synthetic construct
GGGGDDTVY

SEQ ID NO: 46315 - protein, 9 aa, synthetic construct
GGGGDDTYF

SEQ ID NO: 46316 - protein, 9 aa, synthetic construct
GGGGDDTYS

SEQ ID NO: 46317 - protein, 9 aa, synthetic construct
GGGGDDVFA

SEQ ID NO: 46318 - protein, 9 aa, synthetic construct
GGGGDDVFF

SEQ ID NO: 46319 - protein, 9 aa, synthetic construct
GGGGDDVFK

SEQ ID NO: 46320 - protein, 9 aa, synthetic construct
GGGGDDVFL

SEQ ID NO: 46321 - protein, 9 aa, synthetic construct
GGGGDDSMG

SEQ ID NO: 46322 - protein, 9 aa, synthetic construct
GGGGDDSME

SEQ ID NO: 46323 - protein, 9 aa, synthetic construct
GGGGDDSLR

SEQ ID NO: 46324 - protein, 9 aa, synthetic construct
GGGGDDRIH

SEQ ID NO: 46325 - protein, 9 aa, synthetic construct
GGGGDDQLQ

SEQ ID NO: 46326 - protein, 9 aa, synthetic construct
GGGGDDQLR

SEQ ID NO: 46327 - protein, 9 aa, synthetic construct
GGGGDDQLS

SEQ ID NO: 46328 - protein, 9 aa, synthetic construct
GGGGDDQLV

SEQ ID NO: 46329 - protein, 9 aa, synthetic construct
GGGGDDQMS

SEQ ID NO: 46330 - protein, 9 aa, synthetic construct
GGGGDDQMW

SEQ ID NO: 46331 - protein, 9 aa, synthetic construct
GGGGDDQMY

SEQ ID NO: 46332 - protein, 9 aa, synthetic construct
GGGGDDQVE

SEQ ID NO: 46333 - protein, 9 aa, synthetic construct
GGGGDDRFE

SEQ ID NO: 46334 - protein, 9 aa, synthetic construct
GGGGDDRFF

SEQ ID NO: 46335 - protein, 9 aa, synthetic construct
GGGGDDRFG

SEQ ID NO: 46336 - protein, 9 aa, synthetic construct
GGGGDDRFT

SEQ ID NO: 46337 - protein, 9 aa, synthetic construct
GGGGDDRFV

SEQ ID NO: 46338 - protein, 9 aa, synthetic construct
GGGGDDRIM

SEQ ID NO: 46339 - protein, 9 aa, synthetic construct
GGGGDDSIW

SEQ ID NO: 46340 - protein, 9 aa, synthetic construct
GGGGDDRLG

SEQ ID NO: 46341 - protein, 9 aa, synthetic construct
GGGGDDRLR

SEQ ID NO: 46342 - protein, 9 aa, synthetic construct
GGGGDDRME

SEQ ID NO: 46343 - protein, 9 aa, synthetic construct
GGGGDDRMF

SEQ ID NO: 46344 - protein, 9 aa, synthetic construct
GGGGDDRMH

SEQ ID NO: 46345 - protein, 9 aa, synthetic construct
GGGGDDRVE

SEQ ID NO: 46346 - protein, 9 aa, synthetic construct
GGGGDDRVH

SEQ ID NO: 46347 - protein, 9 aa, synthetic construct
GGGGDDRVY

SEQ ID NO: 46348 - protein, 9 aa, synthetic construct
GGGGDDSAD

SEQ ID NO: 46349 - protein, 9 aa, synthetic construct
GGGGDDSIH

SEQ ID NO: 46350 - protein, 9 aa, synthetic construct
GGGGDDSIN

SEQ ID NO: 46351 - protein, 9 aa, synthetic construct
GGGGDDSIR

SEQ ID NO: 46352 - protein, 9 aa, synthetic construct
GGGGDDSIS

SEQ ID NO: 46353 - protein, 9 aa, synthetic construct
GGGGDDVFQ

SEQ ID NO: 46354 - protein, 9 aa, synthetic construct
GGGGDDVIH

SEQ ID NO: 46355 - protein, 9 aa, synthetic construct
GGGGDDVIQ

SEQ ID NO: 46356 - protein, 9 aa, synthetic construct
GGGGEDLFL

SEQ ID NO: 46357 - protein, 9 aa, synthetic construct
GGGGEDALS

SEQ ID NO: 46358 - protein, 9 aa, synthetic construct
GGGGEDALY

SEQ ID NO: 46359 - protein, 9 aa, synthetic construct
GGGGEDDLR

SEQ ID NO: 46360 - protein, 9 aa, synthetic construct
GGGGEDEIL

SEQ ID NO: 46361 - protein, 9 aa, synthetic construct
GGGGEDEMY

SEQ ID NO: 46362 - protein, 9 aa, synthetic construct
GGGGEDFID

SEQ ID NO: 46363 - protein, 9 aa, synthetic construct
GGGGEDFMD

SEQ ID NO: 46364 - protein, 9 aa, synthetic construct
GGGGEDIFK

SEQ ID NO: 46365 - protein, 9 aa, synthetic construct
GGGGEDIFV

SEQ ID NO: 46366 - protein, 9 aa, synthetic construct
GGGGEDILD

SEQ ID NO: 46367 - protein, 9 aa, synthetic construct
GGGGEDILT

SEQ ID NO: 46368 - protein, 9 aa, synthetic construct
GGGGEDKFY

SEQ ID NO: 46369 - protein, 9 aa, synthetic construct
GGGGEDKLN

SEQ ID NO: 46370 - protein, 9 aa, synthetic construct
GGGGEDLLI

SEQ ID NO: 46371 - protein, 9 aa, synthetic construct
GGGGEDALF

SEQ ID NO: 46372 - protein, 9 aa, synthetic construct
GGGGEDLLM

SEQ ID NO: 46373 - protein, 9 aa, synthetic construct
GGGGEDNLL

SEQ ID NO: 46374 - protein, 9 aa, synthetic construct
GGGGEDQIA

SEQ ID NO: 46375 - protein, 9 aa, synthetic construct
GGGGEDQLH

SEQ ID NO: 46376 - protein, 9 aa, synthetic construct
GGGGEDQLN

SEQ ID NO: 46377 - protein, 9 aa, synthetic construct
GGGGEDQLW

SEQ ID NO: 46378 - protein, 9 aa, synthetic construct
GGGGEDQMY

SEQ ID NO: 46379 - protein, 9 aa, synthetic construct
GGGGEDRFV

SEQ ID NO: 46380 - protein, 9 aa, synthetic construct
GGGGEDRIW

SEQ ID NO: 46381 - protein, 9 aa, synthetic construct
GGGGEDRLT

SEQ ID NO: 46382 - protein, 9 aa, synthetic construct
GGGGEDRLW

SEQ ID NO: 46383 - protein, 9 aa, synthetic construct
GGGGEDSAM

SEQ ID NO: 46384 - protein, 9 aa, synthetic construct
GGGGEDSFV

SEQ ID NO: 46385 - protein, 9 aa, synthetic construct
GGGGEDALH

SEQ ID NO: 46386 - protein, 9 aa, synthetic construct
GGGGEDAFH

SEQ ID NO: 46387 - protein, 9 aa, synthetic construct
GGGGDDVMH

SEQ ID NO: 46388 - protein, 9 aa, synthetic construct
GGGGDDWVV

SEQ ID NO: 46389 - protein, 9 aa, synthetic construct
GGGGDDVMR

SEQ ID NO: 46390 - protein, 9 aa, synthetic construct
GGGGDDVMV

SEQ ID NO: 46391 - protein, 9 aa, synthetic construct
GGGGDDVVK

SEQ ID NO: 46392 - protein, 9 aa, synthetic construct
GGGGDDVYA

SEQ ID NO: 46393 - protein, 9 aa, synthetic construct
GGGGDDVYR

SEQ ID NO: 46394 - protein, 9 aa, synthetic construct
GGGGDDVYV

SEQ ID NO: 46395 - protein, 9 aa, synthetic construct
GGGGDDVYY

SEQ ID NO: 46396 - protein, 9 aa, synthetic construct
GGGGDDWAA

SEQ ID NO: 46397 - protein, 9 aa, synthetic construct
GGGGDDWFS

SEQ ID NO: 46398 - protein, 9 aa, synthetic construct
GGGGDDWIE

SEQ ID NO: 46399 - protein, 9 aa, synthetic construct
GGGGDDWIK

SEQ ID NO: 46400 - protein, 9 aa, synthetic construct
GGGGDDWLA

SEQ ID NO: 46401 - protein, 9 aa, synthetic construct
GGGGDDWLL

SEQ ID NO: 46402 - protein, 9 aa, synthetic construct
GGGGDDXLS

SEQ ID NO: 46403 - protein, 9 aa, synthetic construct
GGGGDDYVS

SEQ ID NO: 46404 - protein, 9 aa, synthetic construct
GGGGDDYFD

SEQ ID NO: 46405 - protein, 9 aa, synthetic construct
GGGGDDYFF

SEQ ID NO: 46406 - protein, 9 aa, synthetic construct
GGGGDDYII

SEQ ID NO: 46407 - protein, 9 aa, synthetic construct
GGGGDDYIV

SEQ ID NO: 46408 - protein, 9 aa, synthetic construct
GGGGDDYIY

SEQ ID NO: 46409 - protein, 9 aa, synthetic construct
GGGGDDYLC

SEQ ID NO: 46410 - protein, 9 aa, synthetic construct
GGGGDDYLE

SEQ ID NO: 46411 - protein, 9 aa, synthetic construct
GGGGDDYLL

SEQ ID NO: 46412 - protein, 9 aa, synthetic construct
GGGGDDYLN

SEQ ID NO: 46413 - protein, 9 aa, synthetic construct
GGGGDDYLR

SEQ ID NO: 46414 - protein, 9 aa, synthetic construct
GGGGDDYLT

SEQ ID NO: 46415 - protein, 9 aa, synthetic construct
GGGGDDYME

SEQ ID NO: 46416 - protein, 9 aa, synthetic construct
GGGGDDYVD

SEQ ID NO: 46417 - protein, 9 aa, synthetic construct
GGGGDDQLM

SEQ ID NO: 46418 - protein, 9 aa, synthetic construct
GGGGDDQLK

SEQ ID NO: 46419 - protein, 9 aa, synthetic construct
GGGGDDALL

SEQ ID NO: 46420 - protein, 9 aa, synthetic construct
GGGGDDQLI

SEQ ID NO: 46421 - protein, 9 aa, synthetic construct
GGGGDDFID

SEQ ID NO: 46422 - protein, 9 aa, synthetic construct
GGGGDDFIH

SEQ ID NO: 46423 - protein, 9 aa, synthetic construct
GGGGDDFIM

SEQ ID NO: 46424 - protein, 9 aa, synthetic construct
GGGGDDFIN

SEQ ID NO: 46425 - protein, 9 aa, synthetic construct
GGGGDDFIQ

SEQ ID NO: 46426 - protein, 9 aa, synthetic construct
GGGGDDFLD

SEQ ID NO: 46427 - protein, 9 aa, synthetic construct
GGGGDDFMD

SEQ ID NO: 46428 - protein, 9 aa, synthetic construct
GGGGDDFMG

SEQ ID NO: 46429 - protein, 9 aa, synthetic construct
GGGGDDFML

SEQ ID NO: 46430 - protein, 9 aa, synthetic construct
GGGGDDFMS

SEQ ID NO: 46431 - protein, 9 aa, synthetic construct
GGGGDDFVD

SEQ ID NO: 46432 - protein, 9 aa, synthetic construct
GGGGDDFVL

SEQ ID NO: 46433 - protein, 9 aa, synthetic construct
GGGGDDFVS

SEQ ID NO: 46434 - protein, 9 aa, synthetic construct
GGGGDDFVY

SEQ ID NO: 46435 - protein, 9 aa, synthetic construct
GGGGDDFYV

SEQ ID NO: 46436 - protein, 9 aa, synthetic construct
GGGGDDGLA

SEQ ID NO: 46437 - protein, 9 aa, synthetic construct
GGGGDDGLD

SEQ ID NO: 46438 - protein, 9 aa, synthetic construct
GGGGDDGLL

SEQ ID NO: 46439 - protein, 9 aa, synthetic construct
GGGGDDGLR

SEQ ID NO: 46440 - protein, 9 aa, synthetic construct
GGGGDDGLS

SEQ ID NO: 46441 - protein, 9 aa, synthetic construct
GGGGDDGYF

SEQ ID NO: 46442 - protein, 9 aa, synthetic construct
GGGGDDHAH

SEQ ID NO: 46443 - protein, 9 aa, synthetic construct
GGGGDDHAI

SEQ ID NO: 46444 - protein, 9 aa, synthetic construct
GGGGDDHID

SEQ ID NO: 46445 - protein, 9 aa, synthetic construct
GGGGDDHIW

SEQ ID NO: 46446 - protein, 9 aa, synthetic construct
GGGGDDHLE

SEQ ID NO: 46447 - protein, 9 aa, synthetic construct
GGGGDDHLI

SEQ ID NO: 46448 - protein, 9 aa, synthetic construct
GGGGDDHLL

SEQ ID NO: 46449 - protein, 9 aa, synthetic construct
GGGGDDHMH

SEQ ID NO: 46450 - protein, 9 aa, synthetic construct
GGGGDDFIA

SEQ ID NO: 46451 - protein, 9 aa, synthetic construct
GGGGDDEVK

SEQ ID NO: 46452 - protein, 9 aa, synthetic construct
GGGGDDEVI

SEQ ID NO: 46453 - protein, 9 aa, synthetic construct
GGGGDDDLK

SEQ ID NO: 46454 - protein, 9 aa, synthetic construct
GGGGDDALQ

SEQ ID NO: 46455 - protein, 9 aa, synthetic construct
GGGGDDALT

SEQ ID NO: 46456 - protein, 9 aa, synthetic construct
GGGGDDALW

SEQ ID NO: 46457 - protein, 9 aa, synthetic construct
GGGGDDAVV

SEQ ID NO: 46458 - protein, 9 aa, synthetic construct
GGGGDDCID

SEQ ID NO: 46459 - protein, 9 aa, synthetic construct
GGGGDDDAR

SEQ ID NO: 46460 - protein, 9 aa, synthetic construct
GGGGDDDFF

SEQ ID NO: 46461 - protein, 9 aa, synthetic construct
GGGGDDDID

SEQ ID NO: 46462 - protein, 9 aa, synthetic construct
GGGGDDDIL

SEQ ID NO: 46463 - protein, 9 aa, synthetic construct
GGGGDDDIY

SEQ ID NO: 46464 - protein, 9 aa, synthetic construct
GGGGDDDLA

SEQ ID NO: 46465 - protein, 9 aa, synthetic construct
GGGGDDDLH

SEQ ID NO: 46466 - protein, 9 aa, synthetic construct
GGGGDDDLI

SEQ ID NO: 46467 - protein, 9 aa, synthetic construct
GGGGDDDLQ

SEQ ID NO: 46468 - protein, 9 aa, synthetic construct
GGGGDDEVH

SEQ ID NO: 46469 - protein, 9 aa, synthetic construct
GGGGDDDLT

SEQ ID NO: 46470 - protein, 9 aa, synthetic construct
GGGGDDDMD

SEQ ID NO: 46471 - protein, 9 aa, synthetic construct
GGGGDDDME

SEQ ID NO: 46472 - protein, 9 aa, synthetic construct
GGGGDDEAI

SEQ ID NO: 46473 - protein, 9 aa, synthetic construct
GGGGDDEIQ

SEQ ID NO: 46474 - protein, 9 aa, synthetic construct
GGGGDDEIT

SEQ ID NO: 46475 - protein, 9 aa, synthetic construct
GGGGDDELH

SEQ ID NO: 46476 - protein, 9 aa, synthetic construct
GGGGDDELK

SEQ ID NO: 46477 - protein, 9 aa, synthetic construct
GGGGDDELL

SEQ ID NO: 46478 - protein, 9 aa, synthetic construct
GGGGDDELQ

SEQ ID NO: 46479 - protein, 9 aa, synthetic construct
GGGGDDELS

SEQ ID NO: 46480 - protein, 9 aa, synthetic construct
GGGGDDEMS

SEQ ID NO: 46481 - protein, 9 aa, synthetic construct
GGGGDDEVD

SEQ ID NO: 46482 - protein, 9 aa, synthetic construct
GGGGDDHMS

SEQ ID NO: 46483 - protein, 9 aa, synthetic construct
GGGGDDHVW

SEQ ID NO: 46484 - protein, 9 aa, synthetic construct
GGGGDDHVY

SEQ ID NO: 46485 - protein, 9 aa, synthetic construct
GGGGDDMLN

SEQ ID NO: 46486 - protein, 9 aa, synthetic construct
GGGGDDLLC

SEQ ID NO: 46487 - protein, 9 aa, synthetic construct
GGGGDDLLK

SEQ ID NO: 46488 - protein, 9 aa, synthetic construct
GGGGDDLLW

SEQ ID NO: 46489 - protein, 9 aa, synthetic construct
GGGGDDLMT

SEQ ID NO: 46490 - protein, 9 aa, synthetic construct
GGGGDDLYF

SEQ ID NO: 46491 - protein, 9 aa, synthetic construct
GGGGDDLYL

SEQ ID NO: 46492 - protein, 9 aa, synthetic construct
GGGGDDLYR

SEQ ID NO: 46493 - protein, 9 aa, synthetic construct
GGGGDDMAL

SEQ ID NO: 46494 - protein, 9 aa, synthetic construct
GGGGDDMFS

SEQ ID NO: 46495 - protein, 9 aa, synthetic construct
GGGGDDMIE

SEQ ID NO: 46496 - protein, 9 aa, synthetic construct
GGGGDDMIG

SEQ ID NO: 46497 - protein, 9 aa, synthetic construct
GGGGDDMIR

SEQ ID NO: 46498 - protein, 9 aa, synthetic construct
GGGGDDMIS

SEQ ID NO: 46499 - protein, 9 aa, synthetic construct
GGGGDDMMF

SEQ ID NO: 46500 - protein, 9 aa, synthetic construct
GGGGDDLFY

SEQ ID NO: 46501 - protein, 9 aa, synthetic construct
GGGGDDMML

SEQ ID NO: 46502 - protein, 9 aa, synthetic construct
GGGGDDMVD

SEQ ID NO: 46503 - protein, 9 aa, synthetic construct
GGGGDDNID

SEQ ID NO: 46504 - protein, 9 aa, synthetic construct
GGGGDDNLD

SEQ ID NO: 46505 - protein, 9 aa, synthetic construct
GGGGDDNLF

SEQ ID NO: 46506 - protein, 9 aa, synthetic construct
GGGGDDNLQ

SEQ ID NO: 46507 - protein, 9 aa, synthetic construct
GGGGDDNLW

SEQ ID NO: 46508 - protein, 9 aa, synthetic construct
GGGGDDNVN

SEQ ID NO: 46509 - protein, 9 aa, synthetic construct
GGGGDDQAD

SEQ ID NO: 46510 - protein, 9 aa, synthetic construct
GGGGDDQAW

SEQ ID NO: 46511 - protein, 9 aa, synthetic construct
GGGGDDQFV

SEQ ID NO: 46512 - protein, 9 aa, synthetic construct
GGGGDDQIG

SEQ ID NO: 46513 - protein, 9 aa, synthetic construct
GGGGDDQIW

SEQ ID NO: 46514 - protein, 9 aa, synthetic construct
GGGGDDLIC

SEQ ID NO: 46515 - protein, 9 aa, synthetic construct
GGGGDDLFN

SEQ ID NO: 46516 - protein, 9 aa, synthetic construct
GGGGDDIFH

SEQ ID NO: 46517 - protein, 9 aa, synthetic construct
GGGGDDKIE

SEQ ID NO: 46518 - protein, 9 aa, synthetic construct
GGGGDDIFR

SEQ ID NO: 46519 - protein, 9 aa, synthetic construct
GGGGDDIII

SEQ ID NO: 46520 - protein, 9 aa, synthetic construct
GGGGDDIIN

SEQ ID NO: 46521 - protein, 9 aa, synthetic construct
GGGGDDIIS

SEQ ID NO: 46522 - protein, 9 aa, synthetic construct
GGGGDDILY

SEQ ID NO: 46523 - protein, 9 aa, synthetic construct
GGGGDDIVA

SEQ ID NO: 46524 - protein, 9 aa, synthetic construct
GGGGDDIVI

SEQ ID NO: 46525 - protein, 9 aa, synthetic construct
GGGGDDIVS

SEQ ID NO: 46526 - protein, 9 aa, synthetic construct
GGGGDDIYD

SEQ ID NO: 46527 - protein, 9 aa, synthetic construct
GGGGDDIYH

SEQ ID NO: 46528 - protein, 9 aa, synthetic construct
GGGGDDIYL

SEQ ID NO: 46529 - protein, 9 aa, synthetic construct
GGGGDDIYR

SEQ ID NO: 46530 - protein, 9 aa, synthetic construct
GGGGDDIYY

SEQ ID NO: 46531 - protein, 9 aa, synthetic construct
GGGGDDKII

SEQ ID NO: 46532 - protein, 9 aa, synthetic construct
GGGGDDLAM

SEQ ID NO: 46533 - protein, 9 aa, synthetic construct
GGGGDDKIK

SEQ ID NO: 46534 - protein, 9 aa, synthetic construct
GGGGDDKIN

SEQ ID NO: 46535 - protein, 9 aa, synthetic construct
GGGGDDKIS

SEQ ID NO: 46536 - protein, 9 aa, synthetic construct
GGGGDDKIV

SEQ ID NO: 46537 - protein, 9 aa, synthetic construct
GGGGDDKIW

SEQ ID NO: 46538 - protein, 9 aa, synthetic construct
GGGGDDKLH

SEQ ID NO: 46539 - protein, 9 aa, synthetic construct
GGGGDDKLI

SEQ ID NO: 46540 - protein, 9 aa, synthetic construct
GGGGDDKLL

SEQ ID NO: 46541 - protein, 9 aa, synthetic construct
GGGGDDKLN

SEQ ID NO: 46542 - protein, 9 aa, synthetic construct
GGGGDDKLV

SEQ ID NO: 46543 - protein, 9 aa, synthetic construct
GGGGDDKYY

SEQ ID NO: 46544 - protein, 9 aa, synthetic construct
GGGGDDLAF

SEQ ID NO: 46545 - protein, 9 aa, synthetic construct
GGGGDDLAI

SEQ ID NO: 46546 - protein, 9 aa, synthetic construct
GGKGDDAYV

SEQ ID NO: 46547 - protein, 9 aa, synthetic construct
GGKGDDDIY

SEQ ID NO: 46548 - protein, 9 aa, synthetic construct
GGPGDDTIA

SEQ ID NO: 46549 - protein, 9 aa, synthetic construct
GGNGDDIAR

SEQ ID NO: 46550 - protein, 9 aa, synthetic construct
GGNGDDELD

SEQ ID NO: 46551 - protein, 9 aa, synthetic construct
GGNGDDELN

SEQ ID NO: 46552 - protein, 9 aa, synthetic construct
GGNGDDELS

SEQ ID NO: 46553 - protein, 9 aa, synthetic construct
GGNGDDELW

SEQ ID NO: 46554 - protein, 9 aa, synthetic construct
GGNGDDEVD

SEQ ID NO: 46555 - protein, 9 aa, synthetic construct
GGNGDDEVH

SEQ ID NO: 46556 - protein, 9 aa, synthetic construct
GGNGDDEVS

SEQ ID NO: 46557 - protein, 9 aa, synthetic construct
GGNGDDFAA

SEQ ID NO: 46558 - protein, 9 aa, synthetic construct
GGNGDDFAN

SEQ ID NO: 46559 - protein, 9 aa, synthetic construct
GGNGDDFIG

SEQ ID NO: 46560 - protein, 9 aa, synthetic construct
GGNGDDFIR

SEQ ID NO: 46561 - protein, 9 aa, synthetic construct
GGNGDDFIT

SEQ ID NO: 46562 - protein, 9 aa, synthetic construct
GGNGDDFIV

SEQ ID NO: 46563 - protein, 9 aa, synthetic construct
GGNGDDFIW

SEQ ID NO: 46564 - protein, 9 aa, synthetic construct
GGNGDDFLA

SEQ ID NO: 46565 - protein, 9 aa, synthetic construct
GGNGDDFLE

SEQ ID NO: 46566 - protein, 9 aa, synthetic construct
GGNGDDFVL

SEQ ID NO: 46567 - protein, 9 aa, synthetic construct
GGNGDDFVN

SEQ ID NO: 46568 - protein, 9 aa, synthetic construct
GGNGDDGIA

SEQ ID NO: 46569 - protein, 9 aa, synthetic construct
GGNGDDGLL

SEQ ID NO: 46570 - protein, 9 aa, synthetic construct
GGNGDDGLN

SEQ ID NO: 46571 - protein, 9 aa, synthetic construct
GGNGDDGLP

SEQ ID NO: 46572 - protein, 9 aa, synthetic construct
GGNGDDGLT

SEQ ID NO: 46573 - protein, 9 aa, synthetic construct
GGNGDDGYV

SEQ ID NO: 46574 - protein, 9 aa, synthetic construct
GGNGDDHAA

SEQ ID NO: 46575 - protein, 9 aa, synthetic construct
GGNGDDHIH

SEQ ID NO: 46576 - protein, 9 aa, synthetic construct
GGNGDDHLF

SEQ ID NO: 46577 - protein, 9 aa, synthetic construct
GGNGDDHLQ

SEQ ID NO: 46578 - protein, 9 aa, synthetic construct
GGNGDDHMN

SEQ ID NO: 46579 - protein, 9 aa, synthetic construct
GGNGDDEIV

SEQ ID NO: 46580 - protein, 9 aa, synthetic construct
GGNGDDEIT

SEQ ID NO: 46581 - protein, 9 aa, synthetic construct
GGNGDDEIL

SEQ ID NO: 46582 - protein, 9 aa, synthetic construct
GGNGDDCID

SEQ ID NO: 46583 - protein, 9 aa, synthetic construct
GGNGCDLMV

SEQ ID NO: 46584 - protein, 9 aa, synthetic construct
GGNGCDQVW

SEQ ID NO: 46585 - protein, 9 aa, synthetic construct
GGNGCDRLE

SEQ ID NO: 46586 - protein, 9 aa, synthetic construct
GGNGDDAAY

SEQ ID NO: 46587 - protein, 9 aa, synthetic construct
GGNGDDAFE

SEQ ID NO: 46588 - protein, 9 aa, synthetic construct
GGNGDDAFW

SEQ ID NO: 46589 - protein, 9 aa, synthetic construct
GGNGDDAIE

SEQ ID NO: 46590 - protein, 9 aa, synthetic construct
GGNGDDAIG

SEQ ID NO: 46591 - protein, 9 aa, synthetic construct
GGNGDDAIR

SEQ ID NO: 46592 - protein, 9 aa, synthetic construct
GGNGDDAIS

SEQ ID NO: 46593 - protein, 9 aa, synthetic construct
GGNGDDAIY

SEQ ID NO: 46594 - protein, 9 aa, synthetic construct
GGNGDDALV

SEQ ID NO: 46595 - protein, 9 aa, synthetic construct
GGNGDDALY

SEQ ID NO: 46596 - protein, 9 aa, synthetic construct
GGNGDDCLN

SEQ ID NO: 46597 - protein, 9 aa, synthetic construct
GGNGDDDYY

SEQ ID NO: 46598 - protein, 9 aa, synthetic construct
GGNGDDDFD

SEQ ID NO: 46599 - protein, 9 aa, synthetic construct
GGNGDDDFF

SEQ ID NO: 46600 - protein, 9 aa, synthetic construct
GGNGDDDID

SEQ ID NO: 46601 - protein, 9 aa, synthetic construct
GGNGDDDIF

SEQ ID NO: 46602 - protein, 9 aa, synthetic construct
GGNGDDDIR

SEQ ID NO: 46603 - protein, 9 aa, synthetic construct
GGNGDDDIY

SEQ ID NO: 46604 - protein, 9 aa, synthetic construct
GGNGDDDLA

SEQ ID NO: 46605 - protein, 9 aa, synthetic construct
GGNGDDDLD

SEQ ID NO: 46606 - protein, 9 aa, synthetic construct
GGNGDDDLH

SEQ ID NO: 46607 - protein, 9 aa, synthetic construct
GGNGDDDLV

SEQ ID NO: 46608 - protein, 9 aa, synthetic construct
GGNGDDDLY

SEQ ID NO: 46609 - protein, 9 aa, synthetic construct
GGNGDDDMF

SEQ ID NO: 46610 - protein, 9 aa, synthetic construct
GGNGDDDMN

SEQ ID NO: 46611 - protein, 9 aa, synthetic construct
GGNGDDHVR

SEQ ID NO: 46612 - protein, 9 aa, synthetic construct
GGNGDDIAV

SEQ ID NO: 46613 - protein, 9 aa, synthetic construct
GGNGDDQIW

SEQ ID NO: 46614 - protein, 9 aa, synthetic construct
GGNGDDIFI

SEQ ID NO: 46615 - protein, 9 aa, synthetic construct
GGNGDDLMQ

SEQ ID NO: 46616 - protein, 9 aa, synthetic construct
GGNGDDLMT

SEQ ID NO: 46617 - protein, 9 aa, synthetic construct
GGNGDDLVA

SEQ ID NO: 46618 - protein, 9 aa, synthetic construct
GGNGDDLYI

SEQ ID NO: 46619 - protein, 9 aa, synthetic construct
GGNGDDMIA

SEQ ID NO: 46620 - protein, 9 aa, synthetic construct
GGNGDDMII

SEQ ID NO: 46621 - protein, 9 aa, synthetic construct
GGNGDDMIR

SEQ ID NO: 46622 - protein, 9 aa, synthetic construct
GGNGDDMIT

SEQ ID NO: 46623 - protein, 9 aa, synthetic construct
GGNGDDMLD

SEQ ID NO: 46624 - protein, 9 aa, synthetic construct
GGNGDDMLF

SEQ ID NO: 46625 - protein, 9 aa, synthetic construct
GGNGDDMLL

SEQ ID NO: 46626 - protein, 9 aa, synthetic construct
GGNGDDMLM

SEQ ID NO: 46627 - protein, 9 aa, synthetic construct
GGNGDDMML

SEQ ID NO: 46628 - protein, 9 aa, synthetic construct
GGNGDDNAF

SEQ ID NO: 46629 - protein, 9 aa, synthetic construct
GGNGDDNIA

SEQ ID NO: 46630 - protein, 9 aa, synthetic construct
GGNGDDNIN

SEQ ID NO: 46631 - protein, 9 aa, synthetic construct
GGNGDDNIT

SEQ ID NO: 46632 - protein, 9 aa, synthetic construct
GGNGDDNLA

SEQ ID NO: 46633 - protein, 9 aa, synthetic construct
GGNGDDNLD

SEQ ID NO: 46634 - protein, 9 aa, synthetic construct
GGNGDDNLI

SEQ ID NO: 46635 - protein, 9 aa, synthetic construct
GGNGDDNLR

SEQ ID NO: 46636 - protein, 9 aa, synthetic construct
GGNGDDNLS

SEQ ID NO: 46637 - protein, 9 aa, synthetic construct
GGNGDDNMD

SEQ ID NO: 46638 - protein, 9 aa, synthetic construct
GGNGDDNMT

SEQ ID NO: 46639 - protein, 9 aa, synthetic construct
GGNGDDNYY

SEQ ID NO: 46640 - protein, 9 aa, synthetic construct
GGNGDDQAI

SEQ ID NO: 46641 - protein, 9 aa, synthetic construct
GGNGDDQFR

SEQ ID NO: 46642 - protein, 9 aa, synthetic construct
GGNGDDQID

SEQ ID NO: 46643 - protein, 9 aa, synthetic construct
GGNGDDQIF

SEQ ID NO: 46644 - protein, 9 aa, synthetic construct
GGNGDDLME

SEQ ID NO: 46645 - protein, 9 aa, synthetic construct
GGNGDDLLW

SEQ ID NO: 46646 - protein, 9 aa, synthetic construct
GGNGDDLIS

SEQ ID NO: 46647 - protein, 9 aa, synthetic construct
GGNGDDIVY

SEQ ID NO: 46648 - protein, 9 aa, synthetic construct
GGNGDDIFR

SEQ ID NO: 46649 - protein, 9 aa, synthetic construct
GGNGDDIIA

SEQ ID NO: 46650 - protein, 9 aa, synthetic construct
GGNGDDIIE

SEQ ID NO: 46651 - protein, 9 aa, synthetic construct
GGNGDDIIF

SEQ ID NO: 46652 - protein, 9 aa, synthetic construct
GGNGDDIIM

SEQ ID NO: 46653 - protein, 9 aa, synthetic construct
GGNGDDIIN

SEQ ID NO: 46654 - protein, 9 aa, synthetic construct
GGNGDDIIV

SEQ ID NO: 46655 - protein, 9 aa, synthetic construct
GGNGDDIVA

SEQ ID NO: 46656 - protein, 9 aa, synthetic construct
GGNGDDIVD

SEQ ID NO: 46657 - protein, 9 aa, synthetic construct
GGNGDDIVF

SEQ ID NO: 46658 - protein, 9 aa, synthetic construct
GGNGDDIVL

SEQ ID NO: 46659 - protein, 9 aa, synthetic construct
GGNGDDIVS

SEQ ID NO: 46660 - protein, 9 aa, synthetic construct
GGNGDDIVT

SEQ ID NO: 46661 - protein, 9 aa, synthetic construct
GGNGDDIYI

SEQ ID NO: 46662 - protein, 9 aa, synthetic construct
GGNGDDLIQ

SEQ ID NO: 46663 - protein, 9 aa, synthetic construct
GGNGDDIYV

SEQ ID NO: 46664 - protein, 9 aa, synthetic construct
GGNGDDKFT

SEQ ID NO: 46665 - protein, 9 aa, synthetic construct
GGNGDDKID

SEQ ID NO: 46666 - protein, 9 aa, synthetic construct
GGNGDDKIF

SEQ ID NO: 46667 - protein, 9 aa, synthetic construct
GGNGDDKIR

SEQ ID NO: 46668 - protein, 9 aa, synthetic construct
GGNGDDKIY

SEQ ID NO: 46669 - protein, 9 aa, synthetic construct
GGNGDDKLA

SEQ ID NO: 46670 - protein, 9 aa, synthetic construct
GGNGDDKLH

SEQ ID NO: 46671 - protein, 9 aa, synthetic construct
GGNGDDKLL

SEQ ID NO: 46672 - protein, 9 aa, synthetic construct
GGNGDDKVD

SEQ ID NO: 46673 - protein, 9 aa, synthetic construct
GGNGDDKVK

SEQ ID NO: 46674 - protein, 9 aa, synthetic construct
GGNGDDLAW

SEQ ID NO: 46675 - protein, 9 aa, synthetic construct
GGNGDDLIK

SEQ ID NO: 46676 - protein, 9 aa, synthetic construct
GGNGCDLMI

SEQ ID NO: 46677 - protein, 9 aa, synthetic construct
GGNGCDILF

SEQ ID NO: 46678 - protein, 9 aa, synthetic construct
GGNGADYVN

SEQ ID NO: 46679 - protein, 9 aa, synthetic construct
GGNGADYVD

SEQ ID NO: 46680 - protein, 9 aa, synthetic construct
GGNGADQFM

SEQ ID NO: 46681 - protein, 9 aa, synthetic construct
GGNGADQFV

SEQ ID NO: 46682 - protein, 9 aa, synthetic construct
GGNGADQIE

SEQ ID NO: 46683 - protein, 9 aa, synthetic construct
GGNGADQIS

SEQ ID NO: 46684 - protein, 9 aa, synthetic construct
GGNGADQIY

SEQ ID NO: 46685 - protein, 9 aa, synthetic construct
GGNGADQLA

SEQ ID NO: 46686 - protein, 9 aa, synthetic construct
GGNGADQMD

SEQ ID NO: 46687 - protein, 9 aa, synthetic construct
GGNGADQVR

SEQ ID NO: 46688 - protein, 9 aa, synthetic construct
GGNGADRAT

SEQ ID NO: 46689 - protein, 9 aa, synthetic construct
GGNGADRFQ

SEQ ID NO: 46690 - protein, 9 aa, synthetic construct
GGNGADRFY

SEQ ID NO: 46691 - protein, 9 aa, synthetic construct
GGNGADRIA

SEQ ID NO: 46692 - protein, 9 aa, synthetic construct
GGNGADRIG

SEQ ID NO: 46693 - protein, 9 aa, synthetic construct
GGNGADRII

SEQ ID NO: 46694 - protein, 9 aa, synthetic construct
GGNGADRIS

SEQ ID NO: 46695 - protein, 9 aa, synthetic construct
GGNGADRLM

SEQ ID NO: 46696 - protein, 9 aa, synthetic construct
GGNGADRLQ

SEQ ID NO: 46697 - protein, 9 aa, synthetic construct
GGNGADRMF

SEQ ID NO: 46698 - protein, 9 aa, synthetic construct
GGNGADRMR

SEQ ID NO: 46699 - protein, 9 aa, synthetic construct
GGNGADRMV

SEQ ID NO: 46700 - protein, 9 aa, synthetic construct
GGNGADRVD

SEQ ID NO: 46701 - protein, 9 aa, synthetic construct
GGNGADRVR

SEQ ID NO: 46702 - protein, 9 aa, synthetic construct
GGNGADRVS

SEQ ID NO: 46703 - protein, 9 aa, synthetic construct
GGNGADRVY

SEQ ID NO: 46704 - protein, 9 aa, synthetic construct
GGNGADSFI

SEQ ID NO: 46705 - protein, 9 aa, synthetic construct
GGNGADSFN

SEQ ID NO: 46706 - protein, 9 aa, synthetic construct
GGNGADSFV

SEQ ID NO: 46707 - protein, 9 aa, synthetic construct
GGNGADSIA

SEQ ID NO: 46708 - protein, 9 aa, synthetic construct
GGNGADSIE

SEQ ID NO: 46709 - protein, 9 aa, synthetic construct
GGNGADQFK

SEQ ID NO: 46710 - protein, 9 aa, synthetic construct
GGNGADNMA

SEQ ID NO: 46711 - protein, 9 aa, synthetic construct
GGNGADNLQ

SEQ ID NO: 46712 - protein, 9 aa, synthetic construct
GGNGADLIT

SEQ ID NO: 46713 - protein, 9 aa, synthetic construct
GGNGADILE

SEQ ID NO: 46714 - protein, 9 aa, synthetic construct
GGNGADILK

SEQ ID NO: 46715 - protein, 9 aa, synthetic construct
GGNGADILM

SEQ ID NO: 46716 - protein, 9 aa, synthetic construct
GGNGADIMN

SEQ ID NO: 46717 - protein, 9 aa, synthetic construct
GGNGADIVS

SEQ ID NO: 46718 - protein, 9 aa, synthetic construct
GGNGADIYV

SEQ ID NO: 46719 - protein, 9 aa, synthetic construct
GGNGADKIW

SEQ ID NO: 46720 - protein, 9 aa, synthetic construct
GGNGADKLA

SEQ ID NO: 46721 - protein, 9 aa, synthetic construct
GGNGADLID

SEQ ID NO: 46722 - protein, 9 aa, synthetic construct
GGNGADLIF

SEQ ID NO: 46723 - protein, 9 aa, synthetic construct
GGNGADLII

SEQ ID NO: 46724 - protein, 9 aa, synthetic construct
GGNGADLIR

SEQ ID NO: 46725 - protein, 9 aa, synthetic construct
GGNGADLIS

SEQ ID NO: 46726 - protein, 9 aa, synthetic construct
GGNGADLIV

SEQ ID NO: 46727 - protein, 9 aa, synthetic construct
GGNGADNLK

SEQ ID NO: 46728 - protein, 9 aa, synthetic construct
GGNGADLIW

SEQ ID NO: 46729 - protein, 9 aa, synthetic construct
GGNGADLLH

SEQ ID NO: 46730 - protein, 9 aa, synthetic construct
GGNGADLLM

SEQ ID NO: 46731 - protein, 9 aa, synthetic construct
GGNGADLMQ

SEQ ID NO: 46732 - protein, 9 aa, synthetic construct
GGNGADLMT

SEQ ID NO: 46733 - protein, 9 aa, synthetic construct
GGNGADLMV

SEQ ID NO: 46734 - protein, 9 aa, synthetic construct
GGNGADLYM

SEQ ID NO: 46735 - protein, 9 aa, synthetic construct
GGNGADMFV

SEQ ID NO: 46736 - protein, 9 aa, synthetic construct
GGNGADMIN

SEQ ID NO: 46737 - protein, 9 aa, synthetic construct
GGNGADMLL

SEQ ID NO: 46738 - protein, 9 aa, synthetic construct
GGNGADMLV

SEQ ID NO: 46739 - protein, 9 aa, synthetic construct
GGNGADMLY

SEQ ID NO: 46740 - protein, 9 aa, synthetic construct
GGNGADNIN

SEQ ID NO: 46741 - protein, 9 aa, synthetic construct
GGNGADSIF

SEQ ID NO: 46742 - protein, 9 aa, synthetic construct
GGNGADSII

SEQ ID NO: 46743 - protein, 9 aa, synthetic construct
GGNGADSIQ

SEQ ID NO: 46744 - protein, 9 aa, synthetic construct
GGNGADVYE

SEQ ID NO: 46745 - protein, 9 aa, synthetic construct
GGNGADVFR

SEQ ID NO: 46746 - protein, 9 aa, synthetic construct
GGNGADVII

SEQ ID NO: 46747 - protein, 9 aa, synthetic construct
GGNGADVIM

SEQ ID NO: 46748 - protein, 9 aa, synthetic construct
GGNGADVIS

SEQ ID NO: 46749 - protein, 9 aa, synthetic construct
GGNGADVLE

SEQ ID NO: 46750 - protein, 9 aa, synthetic construct
GGNGADVLL

SEQ ID NO: 46751 - protein, 9 aa, synthetic construct
GGNGADVLM

SEQ ID NO: 46752 - protein, 9 aa, synthetic construct
GGNGADVLR

SEQ ID NO: 46753 - protein, 9 aa, synthetic construct
GGNGADVME

SEQ ID NO: 46754 - protein, 9 aa, synthetic construct
GGNGADVMT

SEQ ID NO: 46755 - protein, 9 aa, synthetic construct
GGNGADVMW

SEQ ID NO: 46756 - protein, 9 aa, synthetic construct
GGNGADVVF

SEQ ID NO: 46757 - protein, 9 aa, synthetic construct
GGNGADVVT

SEQ ID NO: 46758 - protein, 9 aa, synthetic construct
GGNGADVYY

SEQ ID NO: 46759 - protein, 9 aa, synthetic construct
GGNGADVFA

SEQ ID NO: 46760 - protein, 9 aa, synthetic construct
GGNGADWIH

SEQ ID NO: 46761 - protein, 9 aa, synthetic construct
GGNGADWLE

SEQ ID NO: 46762 - protein, 9 aa, synthetic construct
GGNGADWLS

SEQ ID NO: 46763 - protein, 9 aa, synthetic construct
GGNGADWLT

SEQ ID NO: 46764 - protein, 9 aa, synthetic construct
GGNGADWME

SEQ ID NO: 46765 - protein, 9 aa, synthetic construct
GGNGADWVQ

SEQ ID NO: 46766 - protein, 9 aa, synthetic construct
GGNGADYIK

SEQ ID NO: 46767 - protein, 9 aa, synthetic construct
GGNGADYIL

SEQ ID NO: 46768 - protein, 9 aa, synthetic construct
GGNGADYIT

SEQ ID NO: 46769 - protein, 9 aa, synthetic construct
GGNGADYIV

SEQ ID NO: 46770 - protein, 9 aa, synthetic construct
GGNGADYLE

SEQ ID NO: 46771 - protein, 9 aa, synthetic construct
GGNGADYLT

SEQ ID NO: 46772 - protein, 9 aa, synthetic construct
GGNGADYMT

SEQ ID NO: 46773 - protein, 9 aa, synthetic construct
GGNGADVFQ

SEQ ID NO: 46774 - protein, 9 aa, synthetic construct
GGNGADVAR

SEQ ID NO: 46775 - protein, 9 aa, synthetic construct
GGNGADSIR

SEQ ID NO: 46776 - protein, 9 aa, synthetic construct
GGNGADTFT

SEQ ID NO: 46777 - protein, 9 aa, synthetic construct
GGNGADSLG

SEQ ID NO: 46778 - protein, 9 aa, synthetic construct
GGNGADSLH

SEQ ID NO: 46779 - protein, 9 aa, synthetic construct
GGNGADSLI

SEQ ID NO: 46780 - protein, 9 aa, synthetic construct
GGNGADSLK

SEQ ID NO: 46781 - protein, 9 aa, synthetic construct
GGNGADSLV

SEQ ID NO: 46782 - protein, 9 aa, synthetic construct
GGNGADSMI

SEQ ID NO: 46783 - protein, 9 aa, synthetic construct
GGNGADSML

SEQ ID NO: 46784 - protein, 9 aa, synthetic construct
GGNGADSMV

SEQ ID NO: 46785 - protein, 9 aa, synthetic construct
GGNGADSMY

SEQ ID NO: 46786 - protein, 9 aa, synthetic construct
GGNGADSVS

SEQ ID NO: 46787 - protein, 9 aa, synthetic construct
GGNGADSYV

SEQ ID NO: 46788 - protein, 9 aa, synthetic construct
GGNGADTFA

SEQ ID NO: 46789 - protein, 9 aa, synthetic construct
GGNGADTFH

SEQ ID NO: 46790 - protein, 9 aa, synthetic construct
GGNGADTIA

SEQ ID NO: 46791 - protein, 9 aa, synthetic construct
GGNGADTYR

SEQ ID NO: 46792 - protein, 9 aa, synthetic construct
GGNGADTIN

SEQ ID NO: 46793 - protein, 9 aa, synthetic construct
GGNGADTIQ

SEQ ID NO: 46794 - protein, 9 aa, synthetic construct
GGNGADTIS

SEQ ID NO: 46795 - protein, 9 aa, synthetic construct
GGNGADTLG

SEQ ID NO: 46796 - protein, 9 aa, synthetic construct
GGNGADTLQ

SEQ ID NO: 46797 - protein, 9 aa, synthetic construct
GGNGADTME

SEQ ID NO: 46798 - protein, 9 aa, synthetic construct
GGNGADTMH

SEQ ID NO: 46799 - protein, 9 aa, synthetic construct
GGNGADTMN

SEQ ID NO: 46800 - protein, 9 aa, synthetic construct
GGNGADTVE

SEQ ID NO: 46801 - protein, 9 aa, synthetic construct
GGNGADTVF

SEQ ID NO: 46802 - protein, 9 aa, synthetic construct
GGNGADTVI

SEQ ID NO: 46803 - protein, 9 aa, synthetic construct
GGNGADTVM

SEQ ID NO: 46804 - protein, 9 aa, synthetic construct
GGNGADTYL

SEQ ID NO: 46805 - protein, 9 aa, synthetic construct
GGNGDDQIH

SEQ ID NO: 46806 - protein, 9 aa, synthetic construct
GGNGDDQLG

SEQ ID NO: 46807 - protein, 9 aa, synthetic construct
GGNGADIIE

SEQ ID NO: 46808 - protein, 9 aa, synthetic construct
GGNGGDNFQ

SEQ ID NO: 46809 - protein, 9 aa, synthetic construct
GGNGFDVAF

SEQ ID NO: 46810 - protein, 9 aa, synthetic construct
GGNGFDVLF

SEQ ID NO: 46811 - protein, 9 aa, synthetic construct
GGNGGDAFC

SEQ ID NO: 46812 - protein, 9 aa, synthetic construct
GGNGGDALF

SEQ ID NO: 46813 - protein, 9 aa, synthetic construct
GGNGGDALL

SEQ ID NO: 46814 - protein, 9 aa, synthetic construct
GGNGGDDLF

SEQ ID NO: 46815 - protein, 9 aa, synthetic construct
GGNGGDEFH

SEQ ID NO: 46816 - protein, 9 aa, synthetic construct
GGNGGDELQ

SEQ ID NO: 46817 - protein, 9 aa, synthetic construct
GGNGGDEVY

SEQ ID NO: 46818 - protein, 9 aa, synthetic construct
GGNGGDFAY

SEQ ID NO: 46819 - protein, 9 aa, synthetic construct
GGNGGDFID

SEQ ID NO: 46820 - protein, 9 aa, synthetic construct
GGNGGDFIS

SEQ ID NO: 46821 - protein, 9 aa, synthetic construct
GGNGGDFVD

SEQ ID NO: 46822 - protein, 9 aa, synthetic construct
GGNGGDGLF

SEQ ID NO: 46823 - protein, 9 aa, synthetic construct
GGNGGDIAR

SEQ ID NO: 46824 - protein, 9 aa, synthetic construct
GGNGGDIIS

SEQ ID NO: 46825 - protein, 9 aa, synthetic construct
GGNGGDILK

SEQ ID NO: 46826 - protein, 9 aa, synthetic construct
GGNGGDILT

SEQ ID NO: 46827 - protein, 9 aa, synthetic construct
GGNGGDIVD

SEQ ID NO: 46828 - protein, 9 aa, synthetic construct
GGNGGDLIS

SEQ ID NO: 46829 - protein, 9 aa, synthetic construct
GGNGGDLIY

SEQ ID NO: 46830 - protein, 9 aa, synthetic construct
GGNGGDLLD

SEQ ID NO: 46831 - protein, 9 aa, synthetic construct
GGNGGDLLE

SEQ ID NO: 46832 - protein, 9 aa, synthetic construct
GGNGGDLLL

SEQ ID NO: 46833 - protein, 9 aa, synthetic construct
GGNGGDLLV

SEQ ID NO: 46834 - protein, 9 aa, synthetic construct
GGNGGDMFR

SEQ ID NO: 46835 - protein, 9 aa, synthetic construct
GGNGGDMID

SEQ ID NO: 46836 - protein, 9 aa, synthetic construct
GGNGGDMLF

SEQ ID NO: 46837 - protein, 9 aa, synthetic construct
GGNGGDMLL

SEQ ID NO: 46838 - protein, 9 aa, synthetic construct
GGNGFDTVS

SEQ ID NO: 46839 - protein, 9 aa, synthetic construct
GGNGFDTVN

SEQ ID NO: 46840 - protein, 9 aa, synthetic construct
GGNGFDTLS

SEQ ID NO: 46841 - protein, 9 aa, synthetic construct
GGNGFDLLE

SEQ ID NO: 46842 - protein, 9 aa, synthetic construct
GGNGFDFAS

SEQ ID NO: 46843 - protein, 9 aa, synthetic construct
GGNGFDFAV

SEQ ID NO: 46844 - protein, 9 aa, synthetic construct
GGNGFDFLW

SEQ ID NO: 46845 - protein, 9 aa, synthetic construct
GGNGFDFME

SEQ ID NO: 46846 - protein, 9 aa, synthetic construct
GGNGFDHIL

SEQ ID NO: 46847 - protein, 9 aa, synthetic construct
GGNGFDIAD

SEQ ID NO: 46848 - protein, 9 aa, synthetic construct
GGNGFDIID

SEQ ID NO: 46849 - protein, 9 aa, synthetic construct
GGNGFDILD

SEQ ID NO: 46850 - protein, 9 aa, synthetic construct
GGNGFDIVS

SEQ ID NO: 46851 - protein, 9 aa, synthetic construct
GGNGFDKIW

SEQ ID NO: 46852 - protein, 9 aa, synthetic construct
GGNGFDKLK

SEQ ID NO: 46853 - protein, 9 aa, synthetic construct
GGNGFDKLV

SEQ ID NO: 46854 - protein, 9 aa, synthetic construct
GGNGFDLFI

SEQ ID NO: 46855 - protein, 9 aa, synthetic construct
GGNGFDLLN

SEQ ID NO: 46856 - protein, 9 aa, synthetic construct
GGNGFDTLQ

SEQ ID NO: 46857 - protein, 9 aa, synthetic construct
GGNGFDLLT

SEQ ID NO: 46858 - protein, 9 aa, synthetic construct
GGNGFDQVD

SEQ ID NO: 46859 - protein, 9 aa, synthetic construct
GGNGFDQVS

SEQ ID NO: 46860 - protein, 9 aa, synthetic construct
GGNGFDRLS

SEQ ID NO: 46861 - protein, 9 aa, synthetic construct
GGNGFDRLY

SEQ ID NO: 46862 - protein, 9 aa, synthetic construct
GGNGFDSLD

SEQ ID NO: 46863 - protein, 9 aa, synthetic construct
GGNGFDSLS

SEQ ID NO: 46864 - protein, 9 aa, synthetic construct
GGNGFDTAL

SEQ ID NO: 46865 - protein, 9 aa, synthetic construct
GGNGFDTID

SEQ ID NO: 46866 - protein, 9 aa, synthetic construct
GGNGFDTIH

SEQ ID NO: 46867 - protein, 9 aa, synthetic construct
GGNGFDTLE

SEQ ID NO: 46868 - protein, 9 aa, synthetic construct
GGNGFDTLI

SEQ ID NO: 46869 - protein, 9 aa, synthetic construct
GGNGFDTLN

SEQ ID NO: 46870 - protein, 9 aa, synthetic construct
GGNGGDMLY

SEQ ID NO: 46871 - protein, 9 aa, synthetic construct
GGNGGDNLE

SEQ ID NO: 46872 - protein, 9 aa, synthetic construct
GGNGDDQLR

SEQ ID NO: 46873 - protein, 9 aa, synthetic construct
GGNGGDNLQ

SEQ ID NO: 46874 - protein, 9 aa, synthetic construct
GGNGGDWLG

SEQ ID NO: 46875 - protein, 9 aa, synthetic construct
GGNGGDWLS

SEQ ID NO: 46876 - protein, 9 aa, synthetic construct
GGNGGDYLS

SEQ ID NO: 46877 - protein, 9 aa, synthetic construct
GGNGGDYLT

SEQ ID NO: 46878 - protein, 9 aa, synthetic construct
GGNGHDALI

SEQ ID NO: 46879 - protein, 9 aa, synthetic construct
GGNGHDDFY

SEQ ID NO: 46880 - protein, 9 aa, synthetic construct
GGNGHDDLF

SEQ ID NO: 46881 - protein, 9 aa, synthetic construct
GGNGHDDLS

SEQ ID NO: 46882 - protein, 9 aa, synthetic construct
GGNGHDDLY

SEQ ID NO: 46883 - protein, 9 aa, synthetic construct
GGNGHDDVN

SEQ ID NO: 46884 - protein, 9 aa, synthetic construct
GGNGHDEIY

SEQ ID NO: 46885 - protein, 9 aa, synthetic construct
GGNGHDELL

SEQ ID NO: 46886 - protein, 9 aa, synthetic construct
GGNGHDFLD

SEQ ID NO: 46887 - protein, 9 aa, synthetic construct
GGNGHDFMT

SEQ ID NO: 46888 - protein, 9 aa, synthetic construct
GGNGHDFVS

SEQ ID NO: 46889 - protein, 9 aa, synthetic construct
GGNGHDGLW

SEQ ID NO: 46890 - protein, 9 aa, synthetic construct
GGNGHDHLA

SEQ ID NO: 46891 - protein, 9 aa, synthetic construct
GGNGHDHLE

SEQ ID NO: 46892 - protein, 9 aa, synthetic construct
GGNGHDHLR

SEQ ID NO: 46893 - protein, 9 aa, synthetic construct
GGNGHDHLS

SEQ ID NO: 46894 - protein, 9 aa, synthetic construct
GGNGHDIAD

SEQ ID NO: 46895 - protein, 9 aa, synthetic construct
GGNGHDILL

SEQ ID NO: 46896 - protein, 9 aa, synthetic construct
GGNGHDILN

SEQ ID NO: 46897 - protein, 9 aa, synthetic construct
GGNGHDILV

SEQ ID NO: 46898 - protein, 9 aa, synthetic construct
GGNGHDKVI

SEQ ID NO: 46899 - protein, 9 aa, synthetic construct
GGNGHDLLE

SEQ ID NO: 46900 - protein, 9 aa, synthetic construct
GGNGHDLLM

SEQ ID NO: 46901 - protein, 9 aa, synthetic construct
GGNGHDLLQ

SEQ ID NO: 46902 - protein, 9 aa, synthetic construct
GGNGHDLLV

SEQ ID NO: 46903 - protein, 9 aa, synthetic construct
GGNGGDWLD

SEQ ID NO: 46904 - protein, 9 aa, synthetic construct
GGNGGDWLA

SEQ ID NO: 46905 - protein, 9 aa, synthetic construct
GGNGGDVLY

SEQ ID NO: 46906 - protein, 9 aa, synthetic construct
GGNGGDTII

SEQ ID NO: 46907 - protein, 9 aa, synthetic construct
GGNGGDNYW

SEQ ID NO: 46908 - protein, 9 aa, synthetic construct
GGNGGDQIY

SEQ ID NO: 46909 - protein, 9 aa, synthetic construct
GGNGGDQLQ

SEQ ID NO: 46910 - protein, 9 aa, synthetic construct
GGNGGDRFV

SEQ ID NO: 46911 - protein, 9 aa, synthetic construct
GGNGGDRIF

SEQ ID NO: 46912 - protein, 9 aa, synthetic construct
GGNGGDRIG

SEQ ID NO: 46913 - protein, 9 aa, synthetic construct
GGNGGDRLA

SEQ ID NO: 46914 - protein, 9 aa, synthetic construct
GGNGGDRLH

SEQ ID NO: 46915 - protein, 9 aa, synthetic construct
GGNGGDRLN

SEQ ID NO: 46916 - protein, 9 aa, synthetic construct
GGNGGDRLY

SEQ ID NO: 46917 - protein, 9 aa, synthetic construct
GGNGGDRVE

SEQ ID NO: 46918 - protein, 9 aa, synthetic construct
GGNGGDSLR

SEQ ID NO: 46919 - protein, 9 aa, synthetic construct
GGNGGDTID

SEQ ID NO: 46920 - protein, 9 aa, synthetic construct
GGNGGDTIL

SEQ ID NO: 46921 - protein, 9 aa, synthetic construct
GGNGGDVLT

SEQ ID NO: 46922 - protein, 9 aa, synthetic construct
GGNGGDTIS

SEQ ID NO: 46923 - protein, 9 aa, synthetic construct
GGNGGDTLA

SEQ ID NO: 46924 - protein, 9 aa, synthetic construct
GGNGGDTLF

SEQ ID NO: 46925 - protein, 9 aa, synthetic construct
GGNGGDTLK

SEQ ID NO: 46926 - protein, 9 aa, synthetic construct
GGNGGDTLN

SEQ ID NO: 46927 - protein, 9 aa, synthetic construct
GGNGGDTLT

SEQ ID NO: 46928 - protein, 9 aa, synthetic construct
GGNGGDTVE

SEQ ID NO: 46929 - protein, 9 aa, synthetic construct
GGNGGDTYR

SEQ ID NO: 46930 - protein, 9 aa, synthetic construct
GGNGGDVFH

SEQ ID NO: 46931 - protein, 9 aa, synthetic construct
GGNGGDVIY

SEQ ID NO: 46932 - protein, 9 aa, synthetic construct
GGNGGDVLH

SEQ ID NO: 46933 - protein, 9 aa, synthetic construct
GGNGGDVLK

SEQ ID NO: 46934 - protein, 9 aa, synthetic construct
GGNGGDVLS

SEQ ID NO: 46935 - protein, 9 aa, synthetic construct
GGNGFDDLI

SEQ ID NO: 46936 - protein, 9 aa, synthetic construct
GGNGFDALS

SEQ ID NO: 46937 - protein, 9 aa, synthetic construct
GGNGEDYLS

SEQ ID NO: 46938 - protein, 9 aa, synthetic construct
GGNGEDYLN

SEQ ID NO: 46939 - protein, 9 aa, synthetic construct
GGNGDDSYL

SEQ ID NO: 46940 - protein, 9 aa, synthetic construct
GGNGDDSYY

SEQ ID NO: 46941 - protein, 9 aa, synthetic construct
GGNGDDTAQ

SEQ ID NO: 46942 - protein, 9 aa, synthetic construct
GGNGDDTAV

SEQ ID NO: 46943 - protein, 9 aa, synthetic construct
GGNGDDTFD

SEQ ID NO: 46944 - protein, 9 aa, synthetic construct
GGNGDDTIH

SEQ ID NO: 46945 - protein, 9 aa, synthetic construct
GGNGDDTMA

SEQ ID NO: 46946 - protein, 9 aa, synthetic construct
GGNGDDTMD

SEQ ID NO: 46947 - protein, 9 aa, synthetic construct
GGNGDDTMG

SEQ ID NO: 46948 - protein, 9 aa, synthetic construct
GGNGDDTMI

SEQ ID NO: 46949 - protein, 9 aa, synthetic construct
GGNGDDTMR

SEQ ID NO: 46950 - protein, 9 aa, synthetic construct
GGNGDDTMT

SEQ ID NO: 46951 - protein, 9 aa, synthetic construct
GGNGDDTMV

SEQ ID NO: 46952 - protein, 9 aa, synthetic construct
GGNGDDTVF

SEQ ID NO: 46953 - protein, 9 aa, synthetic construct
GGNGDDTVG

SEQ ID NO: 46954 - protein, 9 aa, synthetic construct
GGNGDDTVH

SEQ ID NO: 46955 - protein, 9 aa, synthetic construct
GGNGDDTVM

SEQ ID NO: 46956 - protein, 9 aa, synthetic construct
GGNGDDTVY

SEQ ID NO: 46957 - protein, 9 aa, synthetic construct
GGNGDDTYR

SEQ ID NO: 46958 - protein, 9 aa, synthetic construct
GGNGDDVAK

SEQ ID NO: 46959 - protein, 9 aa, synthetic construct
GGNGDDVAS

SEQ ID NO: 46960 - protein, 9 aa, synthetic construct
GGNGDDVFF

SEQ ID NO: 46961 - protein, 9 aa, synthetic construct
GGNGDDVFN

SEQ ID NO: 46962 - protein, 9 aa, synthetic construct
GGNGDDVIA

SEQ ID NO: 46963 - protein, 9 aa, synthetic construct
GGNGDDVII

SEQ ID NO: 46964 - protein, 9 aa, synthetic construct
GGNGDDVIQ

SEQ ID NO: 46965 - protein, 9 aa, synthetic construct
GGNGDDVIS

SEQ ID NO: 46966 - protein, 9 aa, synthetic construct
GGNGDDVIV

SEQ ID NO: 46967 - protein, 9 aa, synthetic construct
GGNGDDVYI

SEQ ID NO: 46968 - protein, 9 aa, synthetic construct
GGNGDDSYI

SEQ ID NO: 46969 - protein, 9 aa, synthetic construct
GGNGDDSVV

SEQ ID NO: 46970 - protein, 9 aa, synthetic construct
GGNGDDSVN

SEQ ID NO: 46971 - protein, 9 aa, synthetic construct
GGNGDDRYV

SEQ ID NO: 46972 - protein, 9 aa, synthetic construct
GGNGDDQLS

SEQ ID NO: 46973 - protein, 9 aa, synthetic construct
GGNGDDQMI

SEQ ID NO: 46974 - protein, 9 aa, synthetic construct
GGNGDDQMN

SEQ ID NO: 46975 - protein, 9 aa, synthetic construct
GGNGDDQMS

SEQ ID NO: 46976 - protein, 9 aa, synthetic construct
GGNGDDQVF

SEQ ID NO: 46977 - protein, 9 aa, synthetic construct
GGNGDDRAH

SEQ ID NO: 46978 - protein, 9 aa, synthetic construct
GGNGDDRFW

SEQ ID NO: 46979 - protein, 9 aa, synthetic construct
GGNGDDRIT

SEQ ID NO: 46980 - protein, 9 aa, synthetic construct
GGNGDDRLW

SEQ ID NO: 46981 - protein, 9 aa, synthetic construct
GGNGDDRMD

SEQ ID NO: 46982 - protein, 9 aa, synthetic construct
GGNGDDRMF

SEQ ID NO: 46983 - protein, 9 aa, synthetic construct
GGNGDDRMI

SEQ ID NO: 46984 - protein, 9 aa, synthetic construct
GGNGDDRML

SEQ ID NO: 46985 - protein, 9 aa, synthetic construct
GGNGDDSAF

SEQ ID NO: 46986 - protein, 9 aa, synthetic construct
GGNGDDSVI

SEQ ID NO: 46987 - protein, 9 aa, synthetic construct
GGNGDDSAV

SEQ ID NO: 46988 - protein, 9 aa, synthetic construct
GGNGDDSFH

SEQ ID NO: 46989 - protein, 9 aa, synthetic construct
GGNGDDSFI

SEQ ID NO: 46990 - protein, 9 aa, synthetic construct
GGNGDDSIA

SEQ ID NO: 46991 - protein, 9 aa, synthetic construct
GGNGDDSIE

SEQ ID NO: 46992 - protein, 9 aa, synthetic construct
GGNGDDSIR

SEQ ID NO: 46993 - protein, 9 aa, synthetic construct
GGNGDDSIS

SEQ ID NO: 46994 - protein, 9 aa, synthetic construct
GGNGDDSLR

SEQ ID NO: 46995 - protein, 9 aa, synthetic construct
GGNGDDSMD

SEQ ID NO: 46996 - protein, 9 aa, synthetic construct
GGNGDDSMS

SEQ ID NO: 46997 - protein, 9 aa, synthetic construct
GGNGDDSMT

SEQ ID NO: 46998 - protein, 9 aa, synthetic construct
GGNGDDSMV

SEQ ID NO: 46999 - protein, 9 aa, synthetic construct
GGNGDDSMY

SEQ ID NO: 47000 - protein, 9 aa, synthetic construct
GGNGDDVYQ

SEQ ID NO: 47001 - protein, 9 aa, synthetic construct
GGNGDDWLA

SEQ ID NO: 47002 - protein, 9 aa, synthetic construct
GGNGDDWLF

SEQ ID NO: 47003 - protein, 9 aa, synthetic construct
GGNGEDTLD

SEQ ID NO: 47004 - protein, 9 aa, synthetic construct
GGNGEDRFI

SEQ ID NO: 47005 - protein, 9 aa, synthetic construct
GGNGEDRLF

SEQ ID NO: 47006 - protein, 9 aa, synthetic construct
GGNGEDRLL

SEQ ID NO: 47007 - protein, 9 aa, synthetic construct
GGNGEDRVI

SEQ ID NO: 47008 - protein, 9 aa, synthetic construct
GGNGEDRVS

SEQ ID NO: 47009 - protein, 9 aa, synthetic construct
GGNGEDTID

SEQ ID NO: 47010 - protein, 9 aa, synthetic construct
GGNGEDTIE

SEQ ID NO: 47011 - protein, 9 aa, synthetic construct
GGNGEDTIH

SEQ ID NO: 47012 - protein, 9 aa, synthetic construct
GGNGEDTII

SEQ ID NO: 47013 - protein, 9 aa, synthetic construct
GGNGEDTIK

SEQ ID NO: 47014 - protein, 9 aa, synthetic construct
GGNGEDTIN

SEQ ID NO: 47015 - protein, 9 aa, synthetic construct
GGNGEDTIT

SEQ ID NO: 47016 - protein, 9 aa, synthetic construct
GGNGEDTIY

SEQ ID NO: 47017 - protein, 9 aa, synthetic construct
GGNGEDTLE

SEQ ID NO: 47018 - protein, 9 aa, synthetic construct
GGNGEDNLI

SEQ ID NO: 47019 - protein, 9 aa, synthetic construct
GGNGEDTLK

SEQ ID NO: 47020 - protein, 9 aa, synthetic construct
GGNGEDTLY

SEQ ID NO: 47021 - protein, 9 aa, synthetic construct
GGNGEDTVF

SEQ ID NO: 47022 - protein, 9 aa, synthetic construct
GGNGEDTVK

SEQ ID NO: 47023 - protein, 9 aa, synthetic construct
GGNGEDTVY

SEQ ID NO: 47024 - protein, 9 aa, synthetic construct
GGNGEDVIA

SEQ ID NO: 47025 - protein, 9 aa, synthetic construct
GGNGEDVLI

SEQ ID NO: 47026 - protein, 9 aa, synthetic construct
GGNGEDVLN

SEQ ID NO: 47027 - protein, 9 aa, synthetic construct
GGNGEDVLS

SEQ ID NO: 47028 - protein, 9 aa, synthetic construct
GGNGEDVLY

SEQ ID NO: 47029 - protein, 9 aa, synthetic construct
GGNGEDWLE

SEQ ID NO: 47030 - protein, 9 aa, synthetic construct
GGNGEDWMV

SEQ ID NO: 47031 - protein, 9 aa, synthetic construct
GGNGEDYLI

SEQ ID NO: 47032 - protein, 9 aa, synthetic construct
GGNGEDNLL

SEQ ID NO: 47033 - protein, 9 aa, synthetic construct
GGNGEDNIS

SEQ ID NO: 47034 - protein, 9 aa, synthetic construct
GGNGDDWLG

SEQ ID NO: 47035 - protein, 9 aa, synthetic construct
GGNGEDALF

SEQ ID NO: 47036 - protein, 9 aa, synthetic construct
GGNGDDWLN

SEQ ID NO: 47037 - protein, 9 aa, synthetic construct
GGNGDDWLR

SEQ ID NO: 47038 - protein, 9 aa, synthetic construct
GGNGDDWLS

SEQ ID NO: 47039 - protein, 9 aa, synthetic construct
GGNGDDWVA

SEQ ID NO: 47040 - protein, 9 aa, synthetic construct
GGNGDDWVY

SEQ ID NO: 47041 - protein, 9 aa, synthetic construct
GGNGDDYAS

SEQ ID NO: 47042 - protein, 9 aa, synthetic construct
GGNGDDYLK

SEQ ID NO: 47043 - protein, 9 aa, synthetic construct
GGNGDDYMS

SEQ ID NO: 47044 - protein, 9 aa, synthetic construct
GGNGDDYVD

SEQ ID NO: 47045 - protein, 9 aa, synthetic construct
GGNGDDYVG

SEQ ID NO: 47046 - protein, 9 aa, synthetic construct
GGNGDDYVI

SEQ ID NO: 47047 - protein, 9 aa, synthetic construct
GGNGDDYYI

SEQ ID NO: 47048 - protein, 9 aa, synthetic construct
GGNGEDAIE

SEQ ID NO: 47049 - protein, 9 aa, synthetic construct
GGNGEDDLY

SEQ ID NO: 47050 - protein, 9 aa, synthetic construct
GGNGEDMMY

SEQ ID NO: 47051 - protein, 9 aa, synthetic construct
GGNGEDELF

SEQ ID NO: 47052 - protein, 9 aa, synthetic construct
GGNGEDELS

SEQ ID NO: 47053 - protein, 9 aa, synthetic construct
GGNGEDELY

SEQ ID NO: 47054 - protein, 9 aa, synthetic construct
GGNGEDFIE

SEQ ID NO: 47055 - protein, 9 aa, synthetic construct
GGNGEDFLF

SEQ ID NO: 47056 - protein, 9 aa, synthetic construct
GGNGEDHFV

SEQ ID NO: 47057 - protein, 9 aa, synthetic construct
GGNGEDIFR

SEQ ID NO: 47058 - protein, 9 aa, synthetic construct
GGNGEDIIF

SEQ ID NO: 47059 - protein, 9 aa, synthetic construct
GGNGEDILK

SEQ ID NO: 47060 - protein, 9 aa, synthetic construct
GGNGEDILR

SEQ ID NO: 47061 - protein, 9 aa, synthetic construct
GGNGEDILS

SEQ ID NO: 47062 - protein, 9 aa, synthetic construct
GGNGEDLIL

SEQ ID NO: 47063 - protein, 9 aa, synthetic construct
GGNGEDLLE

SEQ ID NO: 47064 - protein, 9 aa, synthetic construct
GGNGADIIN

SEQ ID NO: 47065 - protein, 9 aa, synthetic construct
GGNGADIFY

SEQ ID NO: 47066 - protein, 9 aa, synthetic construct
GGKGDDDLF

SEQ ID NO: 47067 - protein, 9 aa, synthetic construct
GGMGADWLF

SEQ ID NO: 47068 - protein, 9 aa, synthetic construct
GGMGADQLT

SEQ ID NO: 47069 - protein, 9 aa, synthetic construct
GGMGADQLV

SEQ ID NO: 47070 - protein, 9 aa, synthetic construct
GGMGADRFF

SEQ ID NO: 47071 - protein, 9 aa, synthetic construct
GGMGADRLE

SEQ ID NO: 47072 - protein, 9 aa, synthetic construct
GGMGADRLQ

SEQ ID NO: 47073 - protein, 9 aa, synthetic construct
GGMGADRMF

SEQ ID NO: 47074 - protein, 9 aa, synthetic construct
GGMGADSFD

SEQ ID NO: 47075 - protein, 9 aa, synthetic construct
GGMGADSLF

SEQ ID NO: 47076 - protein, 9 aa, synthetic construct
GGMGADSLL

SEQ ID NO: 47077 - protein, 9 aa, synthetic construct
GGMGADTFK

SEQ ID NO: 47078 - protein, 9 aa, synthetic construct
GGMGADTFN

SEQ ID NO: 47079 - protein, 9 aa, synthetic construct
GGMGADTFR

SEQ ID NO: 47080 - protein, 9 aa, synthetic construct
GGMGADTFV

SEQ ID NO: 47081 - protein, 9 aa, synthetic construct
GGMGADTIE

SEQ ID NO: 47082 - protein, 9 aa, synthetic construct
GGMGADTLA

SEQ ID NO: 47083 - protein, 9 aa, synthetic construct
GGMGADTLF

SEQ ID NO: 47084 - protein, 9 aa, synthetic construct
GGMGADTLN

SEQ ID NO: 47085 - protein, 9 aa, synthetic construct
GGMGADTLS

SEQ ID NO: 47086 - protein, 9 aa, synthetic construct
GGMGADTLY

SEQ ID NO: 47087 - protein, 9 aa, synthetic construct
GGMGADTML

SEQ ID NO: 47088 - protein, 9 aa, synthetic construct
GGMGADTVL

SEQ ID NO: 47089 - protein, 9 aa, synthetic construct
GGMGADTYW

SEQ ID NO: 47090 - protein, 9 aa, synthetic construct
GGMGADVFH

SEQ ID NO: 47091 - protein, 9 aa, synthetic construct
GGMGADVFR

SEQ ID NO: 47092 - protein, 9 aa, synthetic construct
GGMGADVLK

SEQ ID NO: 47093 - protein, 9 aa, synthetic construct
GGMGADVLN

SEQ ID NO: 47094 - protein, 9 aa, synthetic construct
GGMGADVLR

SEQ ID NO: 47095 - protein, 9 aa, synthetic construct
GGMGADVLY

SEQ ID NO: 47096 - protein, 9 aa, synthetic construct
GGMGADVYR

SEQ ID NO: 47097 - protein, 9 aa, synthetic construct
GGMGADQIY

SEQ ID NO: 47098 - protein, 9 aa, synthetic construct
GGMGADNMQ

SEQ ID NO: 47099 - protein, 9 aa, synthetic construct
GGMGADLLI

SEQ ID NO: 47100 - protein, 9 aa, synthetic construct
GGLGYDWLE

SEQ ID NO: 47101 - protein, 9 aa, synthetic construct
GGLGYDILI

SEQ ID NO: 47102 - protein, 9 aa, synthetic construct
GGLGYDILR

SEQ ID NO: 47103 - protein, 9 aa, synthetic construct
GGLGYDLLI

SEQ ID NO: 47104 - protein, 9 aa, synthetic construct
GGLGYDLLN

SEQ ID NO: 47105 - protein, 9 aa, synthetic construct
GGLGYDSIG

SEQ ID NO: 47106 - protein, 9 aa, synthetic construct
GGLGYDTAS

SEQ ID NO: 47107 - protein, 9 aa, synthetic construct
GGLGYDTIL

SEQ ID NO: 47108 - protein, 9 aa, synthetic construct
GGLGYDTLI

SEQ ID NO: 47109 - protein, 9 aa, synthetic construct
GGLGYDTLT

SEQ ID NO: 47110 - protein, 9 aa, synthetic construct
GGLGYDTLV

SEQ ID NO: 47111 - protein, 9 aa, synthetic construct
GGLGYDVLE

SEQ ID NO: 47112 - protein, 9 aa, synthetic construct
GGLGYDVYV

SEQ ID NO: 47113 - protein, 9 aa, synthetic construct
GGLGYDWLA

SEQ ID NO: 47114 - protein, 9 aa, synthetic construct
GGLGYDYLY

SEQ ID NO: 47115 - protein, 9 aa, synthetic construct
GGMGADLLE

SEQ ID NO: 47116 - protein, 9 aa, synthetic construct
GGMGADAID

SEQ ID NO: 47117 - protein, 9 aa, synthetic construct
GGMGADDIF

SEQ ID NO: 47118 - protein, 9 aa, synthetic construct
GGMGADELI

SEQ ID NO: 47119 - protein, 9 aa, synthetic construct
GGMGADELT

SEQ ID NO: 47120 - protein, 9 aa, synthetic construct
GGMGADFVA

SEQ ID NO: 47121 - protein, 9 aa, synthetic construct
GGMGADILD

SEQ ID NO: 47122 - protein, 9 aa, synthetic construct
GGMGADILE

SEQ ID NO: 47123 - protein, 9 aa, synthetic construct
GGMGADILI

SEQ ID NO: 47124 - protein, 9 aa, synthetic construct
GGMGADILS

SEQ ID NO: 47125 - protein, 9 aa, synthetic construct
GGMGADILT

SEQ ID NO: 47126 - protein, 9 aa, synthetic construct
GGMGADKLI

SEQ ID NO: 47127 - protein, 9 aa, synthetic construct
GGMGADKLY

SEQ ID NO: 47128 - protein, 9 aa, synthetic construct
GGMGADLIN

SEQ ID NO: 47129 - protein, 9 aa, synthetic construct
GGMGADWLA

SEQ ID NO: 47130 - protein, 9 aa, synthetic construct
GGMGDDAFY

SEQ ID NO: 47131 - protein, 9 aa, synthetic construct
GGMGDDVVS

SEQ ID NO: 47132 - protein, 9 aa, synthetic construct
GGMGDDELF

SEQ ID NO: 47133 - protein, 9 aa, synthetic construct
GGMGDDSID

SEQ ID NO: 47134 - protein, 9 aa, synthetic construct
GGMGDDSIY

SEQ ID NO: 47135 - protein, 9 aa, synthetic construct
GGMGDDSLG

SEQ ID NO: 47136 - protein, 9 aa, synthetic construct
GGMGDDSLS

SEQ ID NO: 47137 - protein, 9 aa, synthetic construct
GGMGDDSLT

SEQ ID NO: 47138 - protein, 9 aa, synthetic construct
GGMGDDSLW

SEQ ID NO: 47139 - protein, 9 aa, synthetic construct
GGMGDDTAV

SEQ ID NO: 47140 - protein, 9 aa, synthetic construct
GGMGDDTFM

SEQ ID NO: 47141 - protein, 9 aa, synthetic construct
GGMGDDTFV

SEQ ID NO: 47142 - protein, 9 aa, synthetic construct
GGMGDDTLE

SEQ ID NO: 47143 - protein, 9 aa, synthetic construct
GGMGDDTLQ

SEQ ID NO: 47144 - protein, 9 aa, synthetic construct
GGMGDDTLR

SEQ ID NO: 47145 - protein, 9 aa, synthetic construct
GGMGDDTMD

SEQ ID NO: 47146 - protein, 9 aa, synthetic construct
GGMGDDTMI

SEQ ID NO: 47147 - protein, 9 aa, synthetic construct
GGMGDDTMT

SEQ ID NO: 47148 - protein, 9 aa, synthetic construct
GGMGDDTMV

SEQ ID NO: 47149 - protein, 9 aa, synthetic construct
GGMGDDTMY

SEQ ID NO: 47150 - protein, 9 aa, synthetic construct
GGMGDDTVD

SEQ ID NO: 47151 - protein, 9 aa, synthetic construct
GGMGDDTVI

SEQ ID NO: 47152 - protein, 9 aa, synthetic construct
GGMGDDTYI

SEQ ID NO: 47153 - protein, 9 aa, synthetic construct
GGMGDDTYL

SEQ ID NO: 47154 - protein, 9 aa, synthetic construct
GGMGDDVID

SEQ ID NO: 47155 - protein, 9 aa, synthetic construct
GGMGDDVIF

SEQ ID NO: 47156 - protein, 9 aa, synthetic construct
GGMGDDVLD

SEQ ID NO: 47157 - protein, 9 aa, synthetic construct
GGMGDDVLK

SEQ ID NO: 47158 - protein, 9 aa, synthetic construct
GGMGDDVLN

SEQ ID NO: 47159 - protein, 9 aa, synthetic construct
GGMGDDVLQ

SEQ ID NO: 47160 - protein, 9 aa, synthetic construct
GGMGDDVLY

SEQ ID NO: 47161 - protein, 9 aa, synthetic construct
GGMGDDVMT

SEQ ID NO: 47162 - protein, 9 aa, synthetic construct
GGMGDDRML

SEQ ID NO: 47163 - protein, 9 aa, synthetic construct
GGMGDDRLV

SEQ ID NO: 47164 - protein, 9 aa, synthetic construct
GGMGDDRLR

SEQ ID NO: 47165 - protein, 9 aa, synthetic construct
GGMGDDLLS

SEQ ID NO: 47166 - protein, 9 aa, synthetic construct
GGMGDDEMS

SEQ ID NO: 47167 - protein, 9 aa, synthetic construct
GGMGDDEYF

SEQ ID NO: 47168 - protein, 9 aa, synthetic construct
GGMGDDFLG

SEQ ID NO: 47169 - protein, 9 aa, synthetic construct
GGMGDDIFY

SEQ ID NO: 47170 - protein, 9 aa, synthetic construct
GGMGDDILA

SEQ ID NO: 47171 - protein, 9 aa, synthetic construct
GGMGDDILD

SEQ ID NO: 47172 - protein, 9 aa, synthetic construct
GGMGDDILI

SEQ ID NO: 47173 - protein, 9 aa, synthetic construct
GGMGDDILS

SEQ ID NO: 47174 - protein, 9 aa, synthetic construct
GGMGDDIMR

SEQ ID NO: 47175 - protein, 9 aa, synthetic construct
GGMGDDKLE

SEQ ID NO: 47176 - protein, 9 aa, synthetic construct
GGMGDDLID

SEQ ID NO: 47177 - protein, 9 aa, synthetic construct
GGMGDDLLE

SEQ ID NO: 47178 - protein, 9 aa, synthetic construct
GGMGDDLLF

SEQ ID NO: 47179 - protein, 9 aa, synthetic construct
GGMGDDLLV

SEQ ID NO: 47180 - protein, 9 aa, synthetic construct
GGMGDDRLL

SEQ ID NO: 47181 - protein, 9 aa, synthetic construct
GGMGDDLMQ

SEQ ID NO: 47182 - protein, 9 aa, synthetic construct
GGMGDDLVD

SEQ ID NO: 47183 - protein, 9 aa, synthetic construct
GGMGDDMAD

SEQ ID NO: 47184 - protein, 9 aa, synthetic construct
GGMGDDMLE

SEQ ID NO: 47185 - protein, 9 aa, synthetic construct
GGMGDDNIQ

SEQ ID NO: 47186 - protein, 9 aa, synthetic construct
GGMGDDNLH

SEQ ID NO: 47187 - protein, 9 aa, synthetic construct
GGMGDDNLS

SEQ ID NO: 47188 - protein, 9 aa, synthetic construct
GGMGDDQLT

SEQ ID NO: 47189 - protein, 9 aa, synthetic construct
GGMGDDQLY

SEQ ID NO: 47190 - protein, 9 aa, synthetic construct
GGMGDDQMS

SEQ ID NO: 47191 - protein, 9 aa, synthetic construct
GGMGDDQVI

SEQ ID NO: 47192 - protein, 9 aa, synthetic construct
GGMGDDRAL

SEQ ID NO: 47193 - protein, 9 aa, synthetic construct
GGMGDDRLA

SEQ ID NO: 47194 - protein, 9 aa, synthetic construct
GGLGYDAAD

SEQ ID NO: 47195 - protein, 9 aa, synthetic construct
GGLGXDQLQ

SEQ ID NO: 47196 - protein, 9 aa, synthetic construct
GGLGXDLLX

SEQ ID NO: 47197 - protein, 9 aa, synthetic construct
GGLGWDYVF

SEQ ID NO: 47198 - protein, 9 aa, synthetic construct
GGLGTDSLV

SEQ ID NO: 47199 - protein, 9 aa, synthetic construct
GGLGTDSMI

SEQ ID NO: 47200 - protein, 9 aa, synthetic construct
GGLGTDSML

SEQ ID NO: 47201 - protein, 9 aa, synthetic construct
GGLGTDTAD

SEQ ID NO: 47202 - protein, 9 aa, synthetic construct
GGLGTDTAG

SEQ ID NO: 47203 - protein, 9 aa, synthetic construct
GGLGTDTFD

SEQ ID NO: 47204 - protein, 9 aa, synthetic construct
GGLGTDTFI

SEQ ID NO: 47205 - protein, 9 aa, synthetic construct
GGLGTDTFS

SEQ ID NO: 47206 - protein, 9 aa, synthetic construct
GGLGTDTFY

SEQ ID NO: 47207 - protein, 9 aa, synthetic construct
GGLGTDTIA

SEQ ID NO: 47208 - protein, 9 aa, synthetic construct
GGLGTDTIL

SEQ ID NO: 47209 - protein, 9 aa, synthetic construct
GGLGTDTLF

SEQ ID NO: 47210 - protein, 9 aa, synthetic construct
GGLGTDTLH

SEQ ID NO: 47211 - protein, 9 aa, synthetic construct
GGLGTDTLL

SEQ ID NO: 47212 - protein, 9 aa, synthetic construct
GGLGTDTLM

SEQ ID NO: 47213 - protein, 9 aa, synthetic construct
GGLGTDTLR

SEQ ID NO: 47214 - protein, 9 aa, synthetic construct
GGLGTDTLY

SEQ ID NO: 47215 - protein, 9 aa, synthetic construct
GGLGTDTMV

SEQ ID NO: 47216 - protein, 9 aa, synthetic construct
GGLGTDTVA

SEQ ID NO: 47217 - protein, 9 aa, synthetic construct
GGLGTDTVN

SEQ ID NO: 47218 - protein, 9 aa, synthetic construct
GGLGTDTVV

SEQ ID NO: 47219 - protein, 9 aa, synthetic construct
GGLGTDTYE

SEQ ID NO: 47220 - protein, 9 aa, synthetic construct
GGLGTDVAD

SEQ ID NO: 47221 - protein, 9 aa, synthetic construct
GGLGTDVLK

SEQ ID NO: 47222 - protein, 9 aa, synthetic construct
GGLGTDVLM

SEQ ID NO: 47223 - protein, 9 aa, synthetic construct
GGLGTDVLV

SEQ ID NO: 47224 - protein, 9 aa, synthetic construct
GGLGTDVLY

SEQ ID NO: 47225 - protein, 9 aa, synthetic construct
GGLGTDWLF

SEQ ID NO: 47226 - protein, 9 aa, synthetic construct
GGLGTDYIE

SEQ ID NO: 47227 - protein, 9 aa, synthetic construct
GGLGTDSLL

SEQ ID NO: 47228 - protein, 9 aa, synthetic construct
GGLGTDSLI

SEQ ID NO: 47229 - protein, 9 aa, synthetic construct
GGLGTDSLE

SEQ ID NO: 47230 - protein, 9 aa, synthetic construct
GGLGTDNFT

SEQ ID NO: 47231 - protein, 9 aa, synthetic construct
GGLGTDFLN

SEQ ID NO: 47232 - protein, 9 aa, synthetic construct
GGLGTDIFV

SEQ ID NO: 47233 - protein, 9 aa, synthetic construct
GGLGTDILL

SEQ ID NO: 47234 - protein, 9 aa, synthetic construct
GGLGTDILN

SEQ ID NO: 47235 - protein, 9 aa, synthetic construct
GGLGTDILP

SEQ ID NO: 47236 - protein, 9 aa, synthetic construct
GGLGTDILV

SEQ ID NO: 47237 - protein, 9 aa, synthetic construct
GGLGTDKLF

SEQ ID NO: 47238 - protein, 9 aa, synthetic construct
GGLGTDKLT

SEQ ID NO: 47239 - protein, 9 aa, synthetic construct
GGLGTDLIN

SEQ ID NO: 47240 - protein, 9 aa, synthetic construct
GGLGTDLLE

SEQ ID NO: 47241 - protein, 9 aa, synthetic construct
GGLGTDLLQ

SEQ ID NO: 47242 - protein, 9 aa, synthetic construct
GGLGTDLVY

SEQ ID NO: 47243 - protein, 9 aa, synthetic construct
GGLGTDMIS

SEQ ID NO: 47244 - protein, 9 aa, synthetic construct
GGLGTDNID

SEQ ID NO: 47245 - protein, 9 aa, synthetic construct
GGLGTDSLA

SEQ ID NO: 47246 - protein, 9 aa, synthetic construct
GGLGTDNIF

SEQ ID NO: 47247 - protein, 9 aa, synthetic construct
GGLGTDNLG

SEQ ID NO: 47248 - protein, 9 aa, synthetic construct
GGLGTDNLS

SEQ ID NO: 47249 - protein, 9 aa, synthetic construct
GGLGTDNLT

SEQ ID NO: 47250 - protein, 9 aa, synthetic construct
GGLGTDQFY

SEQ ID NO: 47251 - protein, 9 aa, synthetic construct
GGLGTDQLS

SEQ ID NO: 47252 - protein, 9 aa, synthetic construct
GGLGTDQLT

SEQ ID NO: 47253 - protein, 9 aa, synthetic construct
GGLGTDQMT

SEQ ID NO: 47254 - protein, 9 aa, synthetic construct
GGLGTDQVF

SEQ ID NO: 47255 - protein, 9 aa, synthetic construct
GGLGTDRIF

SEQ ID NO: 47256 - protein, 9 aa, synthetic construct
GGLGTDRLE

SEQ ID NO: 47257 - protein, 9 aa, synthetic construct
GGLGTDRLL

SEQ ID NO: 47258 - protein, 9 aa, synthetic construct
GGLGTDRLY

SEQ ID NO: 47259 - protein, 9 aa, synthetic construct
GGLGTDYIS

SEQ ID NO: 47260 - protein, 9 aa, synthetic construct
GGLGTDYLR

SEQ ID NO: 47261 - protein, 9 aa, synthetic construct
GGLGTDYLS

SEQ ID NO: 47262 - protein, 9 aa, synthetic construct
GGLGVDVLN

SEQ ID NO: 47263 - protein, 9 aa, synthetic construct
GGLGVDTIK

SEQ ID NO: 47264 - protein, 9 aa, synthetic construct
GGLGVDTIT

SEQ ID NO: 47265 - protein, 9 aa, synthetic construct
GGLGVDTLE

SEQ ID NO: 47266 - protein, 9 aa, synthetic construct
GGLGVDTLF

SEQ ID NO: 47267 - protein, 9 aa, synthetic construct
GGLGVDTLQ

SEQ ID NO: 47268 - protein, 9 aa, synthetic construct
GGLGVDTLR

SEQ ID NO: 47269 - protein, 9 aa, synthetic construct
GGLGVDTMM

SEQ ID NO: 47270 - protein, 9 aa, synthetic construct
GGLGVDTMR

SEQ ID NO: 47271 - protein, 9 aa, synthetic construct
GGLGVDTMS

SEQ ID NO: 47272 - protein, 9 aa, synthetic construct
GGLGVDTMY

SEQ ID NO: 47273 - protein, 9 aa, synthetic construct
GGLGVDTVY

SEQ ID NO: 47274 - protein, 9 aa, synthetic construct
GGLGVDTYL

SEQ ID NO: 47275 - protein, 9 aa, synthetic construct
GGLGVDTYV

SEQ ID NO: 47276 - protein, 9 aa, synthetic construct
GGLGVDVLY

SEQ ID NO: 47277 - protein, 9 aa, synthetic construct
GGLGVDTFV

SEQ ID NO: 47278 - protein, 9 aa, synthetic construct
GGLGVDVMT

SEQ ID NO: 47279 - protein, 9 aa, synthetic construct
GGLGVDVVR

SEQ ID NO: 47280 - protein, 9 aa, synthetic construct
GGLGVDWLD

SEQ ID NO: 47281 - protein, 9 aa, synthetic construct
GGLGVDWLQ

SEQ ID NO: 47282 - protein, 9 aa, synthetic construct
GGLGVDYVI

SEQ ID NO: 47283 - protein, 9 aa, synthetic construct
GGLGWDIAS

SEQ ID NO: 47284 - protein, 9 aa, synthetic construct
GGLGWDKLF

SEQ ID NO: 47285 - protein, 9 aa, synthetic construct
GGLGWDLAI

SEQ ID NO: 47286 - protein, 9 aa, synthetic construct
GGLGWDRFE

SEQ ID NO: 47287 - protein, 9 aa, synthetic construct
GGLGWDRVD

SEQ ID NO: 47288 - protein, 9 aa, synthetic construct
GGLGWDSLS

SEQ ID NO: 47289 - protein, 9 aa, synthetic construct
GGLGWDTLD

SEQ ID NO: 47290 - protein, 9 aa, synthetic construct
GGLGWDTLR

SEQ ID NO: 47291 - protein, 9 aa, synthetic construct
GGLGVDTIH

SEQ ID NO: 47292 - protein, 9 aa, synthetic construct
GGLGVDSLW

SEQ ID NO: 47293 - protein, 9 aa, synthetic construct
GGLGVDEML

SEQ ID NO: 47294 - protein, 9 aa, synthetic construct
GGLGVDILF

SEQ ID NO: 47295 - protein, 9 aa, synthetic construct
GGLGVDFAW

SEQ ID NO: 47296 - protein, 9 aa, synthetic construct
GGLGVDFIL

SEQ ID NO: 47297 - protein, 9 aa, synthetic construct
GGLGVDFLG

SEQ ID NO: 47298 - protein, 9 aa, synthetic construct
GGLGVDFLH

SEQ ID NO: 47299 - protein, 9 aa, synthetic construct
GGLGVDFLS

SEQ ID NO: 47300 - protein, 9 aa, synthetic construct
GGLGVDFLT

SEQ ID NO: 47301 - protein, 9 aa, synthetic construct
GGLGVDFLY

SEQ ID NO: 47302 - protein, 9 aa, synthetic construct
GGLGVDHLI

SEQ ID NO: 47303 - protein, 9 aa, synthetic construct
GGLGVDHLL

SEQ ID NO: 47304 - protein, 9 aa, synthetic construct
GGLGVDIFN

SEQ ID NO: 47305 - protein, 9 aa, synthetic construct
GGLGVDIIS

SEQ ID NO: 47306 - protein, 9 aa, synthetic construct
GGLGVDIIT

SEQ ID NO: 47307 - protein, 9 aa, synthetic construct
GGLGVDILD

SEQ ID NO: 47308 - protein, 9 aa, synthetic construct
GGLGVDILT

SEQ ID NO: 47309 - protein, 9 aa, synthetic construct
GGLGVDSLR

SEQ ID NO: 47310 - protein, 9 aa, synthetic construct
GGLGVDIVD

SEQ ID NO: 47311 - protein, 9 aa, synthetic construct
GGLGVDKMI

SEQ ID NO: 47312 - protein, 9 aa, synthetic construct
GGLGVDLID

SEQ ID NO: 47313 - protein, 9 aa, synthetic construct
GGLGVDLLR

SEQ ID NO: 47314 - protein, 9 aa, synthetic construct
GGLGVDLMT

SEQ ID NO: 47315 - protein, 9 aa, synthetic construct
GGLGVDNLR

SEQ ID NO: 47316 - protein, 9 aa, synthetic construct
GGLGVDQIS

SEQ ID NO: 47317 - protein, 9 aa, synthetic construct
GGLGVDRIA

SEQ ID NO: 47318 - protein, 9 aa, synthetic construct
GGLGVDRII

SEQ ID NO: 47319 - protein, 9 aa, synthetic construct
GGLGVDSFI

SEQ ID NO: 47320 - protein, 9 aa, synthetic construct
GGLGVDSLA

SEQ ID NO: 47321 - protein, 9 aa, synthetic construct
GGLGVDSLF

SEQ ID NO: 47322 - protein, 9 aa, synthetic construct
GGLGVDSLI

SEQ ID NO: 47323 - protein, 9 aa, synthetic construct
GGMGDDVVH

SEQ ID NO: 47324 - protein, 9 aa, synthetic construct
GGMGDDWIE

SEQ ID NO: 47325 - protein, 9 aa, synthetic construct
GGNGADIAF

SEQ ID NO: 47326 - protein, 9 aa, synthetic construct
GGMGSDILE

SEQ ID NO: 47327 - protein, 9 aa, synthetic construct
GGMGQDTLT

SEQ ID NO: 47328 - protein, 9 aa, synthetic construct
GGMGQDTVL

SEQ ID NO: 47329 - protein, 9 aa, synthetic construct
GGMGRDDLY

SEQ ID NO: 47330 - protein, 9 aa, synthetic construct
GGMGRDELT

SEQ ID NO: 47331 - protein, 9 aa, synthetic construct
GGMGRDEMA

SEQ ID NO: 47332 - protein, 9 aa, synthetic construct
GGMGRDFMY

SEQ ID NO: 47333 - protein, 9 aa, synthetic construct
GGMGRDHLD

SEQ ID NO: 47334 - protein, 9 aa, synthetic construct
GGMGRDILT

SEQ ID NO: 47335 - protein, 9 aa, synthetic construct
GGMGRDKLF

SEQ ID NO: 47336 - protein, 9 aa, synthetic construct
GGMGRDLLA

SEQ ID NO: 47337 - protein, 9 aa, synthetic construct
GGMGRDRLA

SEQ ID NO: 47338 - protein, 9 aa, synthetic construct
GGMGRDRLF

SEQ ID NO: 47339 - protein, 9 aa, synthetic construct
GGMGRDTFR

SEQ ID NO: 47340 - protein, 9 aa, synthetic construct
GGMGRDTIL

SEQ ID NO: 47341 - protein, 9 aa, synthetic construct
GGMGRDTLS

SEQ ID NO: 47342 - protein, 9 aa, synthetic construct
GGMGRDTLW

SEQ ID NO: 47343 - protein, 9 aa, synthetic construct
GGMGRDVAD

SEQ ID NO: 47344 - protein, 9 aa, synthetic construct
GGMGRDVFA

SEQ ID NO: 47345 - protein, 9 aa, synthetic construct
GGMGRDVIE

SEQ ID NO: 47346 - protein, 9 aa, synthetic construct
GGMGRDVLS

SEQ ID NO: 47347 - protein, 9 aa, synthetic construct
GGMGRDVLT

SEQ ID NO: 47348 - protein, 9 aa, synthetic construct
GGMGRDVLY

SEQ ID NO: 47349 - protein, 9 aa, synthetic construct
GGMGRDYLA

SEQ ID NO: 47350 - protein, 9 aa, synthetic construct
GGMGSDAFV

SEQ ID NO: 47351 - protein, 9 aa, synthetic construct
GGMGSDDIS

SEQ ID NO: 47352 - protein, 9 aa, synthetic construct
GGMGSDELI

SEQ ID NO: 47353 - protein, 9 aa, synthetic construct
GGMGSDFLL

SEQ ID NO: 47354 - protein, 9 aa, synthetic construct
GGMGSDHIL

SEQ ID NO: 47355 - protein, 9 aa, synthetic construct
GGMGSDHLY

SEQ ID NO: 47356 - protein, 9 aa, synthetic construct
GGMGQDSVY

SEQ ID NO: 47357 - protein, 9 aa, synthetic construct
GGMGQDSLS

SEQ ID NO: 47358 - protein, 9 aa, synthetic construct
GGMGQDRLT

SEQ ID NO: 47359 - protein, 9 aa, synthetic construct
GGMGNDVLW

SEQ ID NO: 47360 - protein, 9 aa, synthetic construct
GGMGNDTME

SEQ ID NO: 47361 - protein, 9 aa, synthetic construct
GGMGNDTMT

SEQ ID NO: 47362 - protein, 9 aa, synthetic construct
GGMGNDTYI

SEQ ID NO: 47363 - protein, 9 aa, synthetic construct
GGMGNDTYL

SEQ ID NO: 47364 - protein, 9 aa, synthetic construct
GGMGNDTYM

SEQ ID NO: 47365 - protein, 9 aa, synthetic construct
GGMGNDTYN

SEQ ID NO: 47366 - protein, 9 aa, synthetic construct
GGMGNDTYS

SEQ ID NO: 47367 - protein, 9 aa, synthetic construct
GGMGNDTYT

SEQ ID NO: 47368 - protein, 9 aa, synthetic construct
GGMGNDVFW

SEQ ID NO: 47369 - protein, 9 aa, synthetic construct
GGMGNDVII

SEQ ID NO: 47370 - protein, 9 aa, synthetic construct
GGMGNDVLA

SEQ ID NO: 47371 - protein, 9 aa, synthetic construct
GGMGNDVLK

SEQ ID NO: 47372 - protein, 9 aa, synthetic construct
GGMGNDVLN

SEQ ID NO: 47373 - protein, 9 aa, synthetic construct
GGMGNDVMQ

SEQ ID NO: 47374 - protein, 9 aa, synthetic construct
GGMGQDRLL

SEQ ID NO: 47375 - protein, 9 aa, synthetic construct
GGMGNDVYY

SEQ ID NO: 47376 - protein, 9 aa, synthetic construct
GGMGNDWIE

SEQ ID NO: 47377 - protein, 9 aa, synthetic construct
GGMGNDWLF

SEQ ID NO: 47378 - protein, 9 aa, synthetic construct
GGMGNDWLI

SEQ ID NO: 47379 - protein, 9 aa, synthetic construct
GGMGNDYLE

SEQ ID NO: 47380 - protein, 9 aa, synthetic construct
GGMGNDYLV

SEQ ID NO: 47381 - protein, 9 aa, synthetic construct
GGMGPDVLL

SEQ ID NO: 47382 - protein, 9 aa, synthetic construct
GGMGQDHLV

SEQ ID NO: 47383 - protein, 9 aa, synthetic construct
GGMGQDILT

SEQ ID NO: 47384 - protein, 9 aa, synthetic construct
GGMGQDQLY

SEQ ID NO: 47385 - protein, 9 aa, synthetic construct
GGMGQDRFW

SEQ ID NO: 47386 - protein, 9 aa, synthetic construct
GGMGQDRIS

SEQ ID NO: 47387 - protein, 9 aa, synthetic construct
GGMGQDRLH

SEQ ID NO: 47388 - protein, 9 aa, synthetic construct
GGMGSDIFY

SEQ ID NO: 47389 - protein, 9 aa, synthetic construct
GGMGSDKLY

SEQ ID NO: 47390 - protein, 9 aa, synthetic construct
GGMGDDWIN

SEQ ID NO: 47391 - protein, 9 aa, synthetic construct
GGMGSDNIT

SEQ ID NO: 47392 - protein, 9 aa, synthetic construct
GGMGYDVMR

SEQ ID NO: 47393 - protein, 9 aa, synthetic construct
GGNGADAFD

SEQ ID NO: 47394 - protein, 9 aa, synthetic construct
GGNGADAIN

SEQ ID NO: 47395 - protein, 9 aa, synthetic construct
GGNGADALI

SEQ ID NO: 47396 - protein, 9 aa, synthetic construct
GGNGADALN

SEQ ID NO: 47397 - protein, 9 aa, synthetic construct
GGNGADALS

SEQ ID NO: 47398 - protein, 9 aa, synthetic construct
GGNGADAYL

SEQ ID NO: 47399 - protein, 9 aa, synthetic construct
GGNGADDFF

SEQ ID NO: 47400 - protein, 9 aa, synthetic construct
GGNGADDLD

SEQ ID NO: 47401 - protein, 9 aa, synthetic construct
GGNGADDLT

SEQ ID NO: 47402 - protein, 9 aa, synthetic construct
GGNGADEAA

SEQ ID NO: 47403 - protein, 9 aa, synthetic construct
GGNGADEIF

SEQ ID NO: 47404 - protein, 9 aa, synthetic construct
GGNGADEIR

SEQ ID NO: 47405 - protein, 9 aa, synthetic construct
GGNGADELF

SEQ ID NO: 47406 - protein, 9 aa, synthetic construct
GGNGADELI

SEQ ID NO: 47407 - protein, 9 aa, synthetic construct
GGNGADEMQ

SEQ ID NO: 47408 - protein, 9 aa, synthetic construct
GGNGADFID

SEQ ID NO: 47409 - protein, 9 aa, synthetic construct
GGNGADFIF

SEQ ID NO: 47410 - protein, 9 aa, synthetic construct
GGNGADFII

SEQ ID NO: 47411 - protein, 9 aa, synthetic construct
GGNGADFIT

SEQ ID NO: 47412 - protein, 9 aa, synthetic construct
GGNGADFIV

SEQ ID NO: 47413 - protein, 9 aa, synthetic construct
GGNGADFLA

SEQ ID NO: 47414 - protein, 9 aa, synthetic construct
GGNGADFLI

SEQ ID NO: 47415 - protein, 9 aa, synthetic construct
GGNGADGMI

SEQ ID NO: 47416 - protein, 9 aa, synthetic construct
GGNGADHFD

SEQ ID NO: 47417 - protein, 9 aa, synthetic construct
GGNGADHFV

SEQ ID NO: 47418 - protein, 9 aa, synthetic construct
GGNGADHLI

SEQ ID NO: 47419 - protein, 9 aa, synthetic construct
GGNGADHLR

SEQ ID NO: 47420 - protein, 9 aa, synthetic construct
GGNGADHLS

SEQ ID NO: 47421 - protein, 9 aa, synthetic construct
GGMGYDTYV

SEQ ID NO: 47422 - protein, 9 aa, synthetic construct
GGMGYDSLD

SEQ ID NO: 47423 - protein, 9 aa, synthetic construct
GGMGWDSLN

SEQ ID NO: 47424 - protein, 9 aa, synthetic construct
GGMGSDTYI

SEQ ID NO: 47425 - protein, 9 aa, synthetic construct
GGMGSDNLA

SEQ ID NO: 47426 - protein, 9 aa, synthetic construct
GGMGSDNLD

SEQ ID NO: 47427 - protein, 9 aa, synthetic construct
GGMGSDRLL

SEQ ID NO: 47428 - protein, 9 aa, synthetic construct
GGMGSDRLS

SEQ ID NO: 47429 - protein, 9 aa, synthetic construct
GGMGSDRYI

SEQ ID NO: 47430 - protein, 9 aa, synthetic construct
GGMGSDSMR

SEQ ID NO: 47431 - protein, 9 aa, synthetic construct
GGMGSDSMS

SEQ ID NO: 47432 - protein, 9 aa, synthetic construct
GGMGSDTIF

SEQ ID NO: 47433 - protein, 9 aa, synthetic construct
GGMGSDTLD

SEQ ID NO: 47434 - protein, 9 aa, synthetic construct
GGMGSDTLK

SEQ ID NO: 47435 - protein, 9 aa, synthetic construct
GGMGSDTLV

SEQ ID NO: 47436 - protein, 9 aa, synthetic construct
GGMGSDTMA

SEQ ID NO: 47437 - protein, 9 aa, synthetic construct
GGMGSDTVR

SEQ ID NO: 47438 - protein, 9 aa, synthetic construct
GGMGTDLFT

SEQ ID NO: 47439 - protein, 9 aa, synthetic construct
GGMGVDVVN

SEQ ID NO: 47440 - protein, 9 aa, synthetic construct
GGMGTDQLN

SEQ ID NO: 47441 - protein, 9 aa, synthetic construct
GGMGTDSLY

SEQ ID NO: 47442 - protein, 9 aa, synthetic construct
GGMGTDTAS

SEQ ID NO: 47443 - protein, 9 aa, synthetic construct
GGMGTDTLD

SEQ ID NO: 47444 - protein, 9 aa, synthetic construct
GGMGTDTLR

SEQ ID NO: 47445 - protein, 9 aa, synthetic construct
GGMGTDTMT

SEQ ID NO: 47446 - protein, 9 aa, synthetic construct
GGMGTDVLQ

SEQ ID NO: 47447 - protein, 9 aa, synthetic construct
GGMGTDVLT

SEQ ID NO: 47448 - protein, 9 aa, synthetic construct
GGMGTDVMS

SEQ ID NO: 47449 - protein, 9 aa, synthetic construct
GGMGVDQMS

SEQ ID NO: 47450 - protein, 9 aa, synthetic construct
GGMGVDTLH

SEQ ID NO: 47451 - protein, 9 aa, synthetic construct
GGMGVDTLV

SEQ ID NO: 47452 - protein, 9 aa, synthetic construct
GGMGVDTMD

SEQ ID NO: 47453 - protein, 9 aa, synthetic construct
GGMGNDTMD

SEQ ID NO: 47454 - protein, 9 aa, synthetic construct
GGMGNDTLM

SEQ ID NO: 47455 - protein, 9 aa, synthetic construct
GGMGNDTLH

SEQ ID NO: 47456 - protein, 9 aa, synthetic construct
GGMGNDTLE

SEQ ID NO: 47457 - protein, 9 aa, synthetic construct
GGMGGDTLL

SEQ ID NO: 47458 - protein, 9 aa, synthetic construct
GGMGGDTLR

SEQ ID NO: 47459 - protein, 9 aa, synthetic construct
GGMGGDWID

SEQ ID NO: 47460 - protein, 9 aa, synthetic construct
GGMGHDAFV

SEQ ID NO: 47461 - protein, 9 aa, synthetic construct
GGMGHDLME

SEQ ID NO: 47462 - protein, 9 aa, synthetic construct
GGMGHDMLT

SEQ ID NO: 47463 - protein, 9 aa, synthetic construct
GGMGHDQLL

SEQ ID NO: 47464 - protein, 9 aa, synthetic construct
GGMGHDSID

SEQ ID NO: 47465 - protein, 9 aa, synthetic construct
GGMGHDSLN

SEQ ID NO: 47466 - protein, 9 aa, synthetic construct
GGMGHDTFR

SEQ ID NO: 47467 - protein, 9 aa, synthetic construct
GGMGHDTIT

SEQ ID NO: 47468 - protein, 9 aa, synthetic construct
GGMGHDTLL

SEQ ID NO: 47469 - protein, 9 aa, synthetic construct
GGMGHDTYV

SEQ ID NO: 47470 - protein, 9 aa, synthetic construct
GGMGIDIID

SEQ ID NO: 47471 - protein, 9 aa, synthetic construct
GGMGIDKLK

SEQ ID NO: 47472 - protein, 9 aa, synthetic construct
GGMGIDLIF

SEQ ID NO: 47473 - protein, 9 aa, synthetic construct
GGMGIDLIT

SEQ ID NO: 47474 - protein, 9 aa, synthetic construct
GGMGIDSMV

SEQ ID NO: 47475 - protein, 9 aa, synthetic construct
GGMGIDTAL

SEQ ID NO: 47476 - protein, 9 aa, synthetic construct
GGMGIDTLK

SEQ ID NO: 47477 - protein, 9 aa, synthetic construct
GGMGIDTLN

SEQ ID NO: 47478 - protein, 9 aa, synthetic construct
GGMGIDVID

SEQ ID NO: 47479 - protein, 9 aa, synthetic construct
GGMGKDALD

SEQ ID NO: 47480 - protein, 9 aa, synthetic construct
GGMGKDILS

SEQ ID NO: 47481 - protein, 9 aa, synthetic construct
GGMGKDMLT

SEQ ID NO: 47482 - protein, 9 aa, synthetic construct
GGMGKDRIV

SEQ ID NO: 47483 - protein, 9 aa, synthetic construct
GGMGKDSIT

SEQ ID NO: 47484 - protein, 9 aa, synthetic construct
GGMGKDSLT

SEQ ID NO: 47485 - protein, 9 aa, synthetic construct
GGMGKDSLY

SEQ ID NO: 47486 - protein, 9 aa, synthetic construct
GGMGGDSYY

SEQ ID NO: 47487 - protein, 9 aa, synthetic construct
GGMGGDSLS

SEQ ID NO: 47488 - protein, 9 aa, synthetic construct
GGMGGDRLL

SEQ ID NO: 47489 - protein, 9 aa, synthetic construct
GGMGEDTLA

SEQ ID NO: 47490 - protein, 9 aa, synthetic construct
GGMGDDWLI

SEQ ID NO: 47491 - protein, 9 aa, synthetic construct
GGMGDDYIL

SEQ ID NO: 47492 - protein, 9 aa, synthetic construct
GGMGDDYLD

SEQ ID NO: 47493 - protein, 9 aa, synthetic construct
GGMGDDYLS

SEQ ID NO: 47494 - protein, 9 aa, synthetic construct
GGMGDDYLY

SEQ ID NO: 47495 - protein, 9 aa, synthetic construct
GGMGEDDLE

SEQ ID NO: 47496 - protein, 9 aa, synthetic construct
GGMGEDELF

SEQ ID NO: 47497 - protein, 9 aa, synthetic construct
GGMGEDHLQ

SEQ ID NO: 47498 - protein, 9 aa, synthetic construct
GGMGEDILV

SEQ ID NO: 47499 - protein, 9 aa, synthetic construct
GGMGEDLLN

SEQ ID NO: 47500 - protein, 9 aa, synthetic construct
GGMGEDQIS

SEQ ID NO: 47501 - protein, 9 aa, synthetic construct
GGMGEDTAS

SEQ ID NO: 47502 - protein, 9 aa, synthetic construct
GGMGEDTFV

SEQ ID NO: 47503 - protein, 9 aa, synthetic construct
GGMGEDTLD

SEQ ID NO: 47504 - protein, 9 aa, synthetic construct
GGMGGDRLD

SEQ ID NO: 47505 - protein, 9 aa, synthetic construct
GGMGEDTLL

SEQ ID NO: 47506 - protein, 9 aa, synthetic construct
GGMGEDTLT

SEQ ID NO: 47507 - protein, 9 aa, synthetic construct
GGMGEDVLI

SEQ ID NO: 47508 - protein, 9 aa, synthetic construct
GGMGEDYIL

SEQ ID NO: 47509 - protein, 9 aa, synthetic construct
GGMGFDIFV

SEQ ID NO: 47510 - protein, 9 aa, synthetic construct
GGMGFDRIF

SEQ ID NO: 47511 - protein, 9 aa, synthetic construct
GGMGFDTLY

SEQ ID NO: 47512 - protein, 9 aa, synthetic construct
GGMGGDDLW

SEQ ID NO: 47513 - protein, 9 aa, synthetic construct
GGMGGDHIY

SEQ ID NO: 47514 - protein, 9 aa, synthetic construct
GGMGGDILD

SEQ ID NO: 47515 - protein, 9 aa, synthetic construct
GGMGGDKLV

SEQ ID NO: 47516 - protein, 9 aa, synthetic construct
GGMGGDLLA

SEQ ID NO: 47517 - protein, 9 aa, synthetic construct
GGMGGDQLS

SEQ ID NO: 47518 - protein, 9 aa, synthetic construct
GGMGKDTIT

SEQ ID NO: 47519 - protein, 9 aa, synthetic construct
GGMGKDTLI

SEQ ID NO: 47520 - protein, 9 aa, synthetic construct
GGMGKDTLS

SEQ ID NO: 47521 - protein, 9 aa, synthetic construct
GGMGNDRLT

SEQ ID NO: 47522 - protein, 9 aa, synthetic construct
GGMGNDLLS

SEQ ID NO: 47523 - protein, 9 aa, synthetic construct
GGMGNDLYR

SEQ ID NO: 47524 - protein, 9 aa, synthetic construct
GGMGNDLYV

SEQ ID NO: 47525 - protein, 9 aa, synthetic construct
GGMGNDMLL

SEQ ID NO: 47526 - protein, 9 aa, synthetic construct
GGMGNDNIN

SEQ ID NO: 47527 - protein, 9 aa, synthetic construct
GGMGNDNLT

SEQ ID NO: 47528 - protein, 9 aa, synthetic construct
GGMGNDQIK

SEQ ID NO: 47529 - protein, 9 aa, synthetic construct
GGMGNDQIS

SEQ ID NO: 47530 - protein, 9 aa, synthetic construct
GGMGNDQLD

SEQ ID NO: 47531 - protein, 9 aa, synthetic construct
GGMGNDQLE

SEQ ID NO: 47532 - protein, 9 aa, synthetic construct
GGMGNDRIS

SEQ ID NO: 47533 - protein, 9 aa, synthetic construct
GGMGNDRLD

SEQ ID NO: 47534 - protein, 9 aa, synthetic construct
GGMGNDRLN

SEQ ID NO: 47535 - protein, 9 aa, synthetic construct
GGMGNDRVE

SEQ ID NO: 47536 - protein, 9 aa, synthetic construct
GGMGNDLLH

SEQ ID NO: 47537 - protein, 9 aa, synthetic construct
GGMGNDSIL

SEQ ID NO: 47538 - protein, 9 aa, synthetic construct
GGMGNDSIV

SEQ ID NO: 47539 - protein, 9 aa, synthetic construct
GGMGNDSLA

SEQ ID NO: 47540 - protein, 9 aa, synthetic construct
GGMGNDSLD

SEQ ID NO: 47541 - protein, 9 aa, synthetic construct
GGMGNDSLE

SEQ ID NO: 47542 - protein, 9 aa, synthetic construct
GGMGNDSLI

SEQ ID NO: 47543 - protein, 9 aa, synthetic construct
GGMGNDSLN

SEQ ID NO: 47544 - protein, 9 aa, synthetic construct
GGMGNDSYI

SEQ ID NO: 47545 - protein, 9 aa, synthetic construct
GGMGNDTFV

SEQ ID NO: 47546 - protein, 9 aa, synthetic construct
GGMGNDTID

SEQ ID NO: 47547 - protein, 9 aa, synthetic construct
GGMGNDTII

SEQ ID NO: 47548 - protein, 9 aa, synthetic construct
GGMGNDTIR

SEQ ID NO: 47549 - protein, 9 aa, synthetic construct
GGMGNDTIV

SEQ ID NO: 47550 - protein, 9 aa, synthetic construct
GGMGNDLLR

SEQ ID NO: 47551 - protein, 9 aa, synthetic construct
GGMGNDLLD

SEQ ID NO: 47552 - protein, 9 aa, synthetic construct
GGMGKDVLV

SEQ ID NO: 47553 - protein, 9 aa, synthetic construct
GGMGNDIAL

SEQ ID NO: 47554 - protein, 9 aa, synthetic construct
GGMGLDILD

SEQ ID NO: 47555 - protein, 9 aa, synthetic construct
GGMGLDRLT

SEQ ID NO: 47556 - protein, 9 aa, synthetic construct
GGMGLDTLT

SEQ ID NO: 47557 - protein, 9 aa, synthetic construct
GGMGNDALK

SEQ ID NO: 47558 - protein, 9 aa, synthetic construct
GGMGNDALY

SEQ ID NO: 47559 - protein, 9 aa, synthetic construct
GGMGNDEAY

SEQ ID NO: 47560 - protein, 9 aa, synthetic construct
GGMGNDELR

SEQ ID NO: 47561 - protein, 9 aa, synthetic construct
GGMGNDELT

SEQ ID NO: 47562 - protein, 9 aa, synthetic construct
GGMGNDFAD

SEQ ID NO: 47563 - protein, 9 aa, synthetic construct
GGMGNDFLN

SEQ ID NO: 47564 - protein, 9 aa, synthetic construct
GGMGNDFVT

SEQ ID NO: 47565 - protein, 9 aa, synthetic construct
GGMGNDGLA

SEQ ID NO: 47566 - protein, 9 aa, synthetic construct
GGMGNDHLF

SEQ ID NO: 47567 - protein, 9 aa, synthetic construct
GGMGNDIIG

SEQ ID NO: 47568 - protein, 9 aa, synthetic construct
GGMGNDLIS

SEQ ID NO: 47569 - protein, 9 aa, synthetic construct
GGMGNDILA

SEQ ID NO: 47570 - protein, 9 aa, synthetic construct
GGMGNDILF

SEQ ID NO: 47571 - protein, 9 aa, synthetic construct
GGMGNDILI

SEQ ID NO: 47572 - protein, 9 aa, synthetic construct
GGMGNDILQ

SEQ ID NO: 47573 - protein, 9 aa, synthetic construct
GGMGNDILR

SEQ ID NO: 47574 - protein, 9 aa, synthetic construct
GGMGNDILS

SEQ ID NO: 47575 - protein, 9 aa, synthetic construct
GGMGNDILT

SEQ ID NO: 47576 - protein, 9 aa, synthetic construct
GGMGNDIVY

SEQ ID NO: 47577 - protein, 9 aa, synthetic construct
GGMGNDIYV

SEQ ID NO: 47578 - protein, 9 aa, synthetic construct
GGMGNDKLV

SEQ ID NO: 47579 - protein, 9 aa, synthetic construct
GGMGNDKLY

SEQ ID NO: 47580 - protein, 9 aa, synthetic construct
GGMGNDLAY

SEQ ID NO: 47581 - protein, 9 aa, synthetic construct
GGMGNDLFR

SEQ ID NO: 47582 - protein, 9 aa, synthetic construct
GGNGHDLMY

SEQ ID NO: 47583 - protein, 9 aa, synthetic construct
GGNGHDNLD

SEQ ID NO: 47584 - protein, 9 aa, synthetic construct
GGNGHDNLI

SEQ ID NO: 47585 - protein, 9 aa, synthetic construct
GGNGTDYLS

SEQ ID NO: 47586 - protein, 9 aa, synthetic construct
GGNGTDLVI

SEQ ID NO: 47587 - protein, 9 aa, synthetic construct
GGNGTDMLL

SEQ ID NO: 47588 - protein, 9 aa, synthetic construct
GGNGTDMLR

SEQ ID NO: 47589 - protein, 9 aa, synthetic construct
GGNGTDNLD

SEQ ID NO: 47590 - protein, 9 aa, synthetic construct
GGNGTDQID

SEQ ID NO: 47591 - protein, 9 aa, synthetic construct
GGNGTDRAF

SEQ ID NO: 47592 - protein, 9 aa, synthetic construct
GGNGTDRLD

SEQ ID NO: 47593 - protein, 9 aa, synthetic construct
GGNGTDSAL

SEQ ID NO: 47594 - protein, 9 aa, synthetic construct
GGNGTDSIT

SEQ ID NO: 47595 - protein, 9 aa, synthetic construct
GGNGTDSLD

SEQ ID NO: 47596 - protein, 9 aa, synthetic construct
GGNGTDSLK

SEQ ID NO: 47597 - protein, 9 aa, synthetic construct
GGNGTDSLS

SEQ ID NO: 47598 - protein, 9 aa, synthetic construct
GGNGTDTAL

SEQ ID NO: 47599 - protein, 9 aa, synthetic construct
GGNGTDTIY

SEQ ID NO: 47600 - protein, 9 aa, synthetic construct
GGNGTDTLE

SEQ ID NO: 47601 - protein, 9 aa, synthetic construct
GGNGTDTLK

SEQ ID NO: 47602 - protein, 9 aa, synthetic construct
GGNGTDTLR

SEQ ID NO: 47603 - protein, 9 aa, synthetic construct
GGNGTDTLS

SEQ ID NO: 47604 - protein, 9 aa, synthetic construct
GGNGTDTLW

SEQ ID NO: 47605 - protein, 9 aa, synthetic construct
GGNGTDTMI

SEQ ID NO: 47606 - protein, 9 aa, synthetic construct
GGNGTDTVE

SEQ ID NO: 47607 - protein, 9 aa, synthetic construct
GGNGTDTVL

SEQ ID NO: 47608 - protein, 9 aa, synthetic construct
GGNGTDTYL

SEQ ID NO: 47609 - protein, 9 aa, synthetic construct
GGNGTDVLL

SEQ ID NO: 47610 - protein, 9 aa, synthetic construct
GGNGTDVLV

SEQ ID NO: 47611 - protein, 9 aa, synthetic construct
GGNGTDVLY

SEQ ID NO: 47612 - protein, 9 aa, synthetic construct
GGNGTDWLD

SEQ ID NO: 47613 - protein, 9 aa, synthetic construct
GGNGTDWVV

SEQ ID NO: 47614 - protein, 9 aa, synthetic construct
GGNGTDYIL

SEQ ID NO: 47615 - protein, 9 aa, synthetic construct
GGNGTDLLY

SEQ ID NO: 47616 - protein, 9 aa, synthetic construct
GGNGTDLLT

SEQ ID NO: 47617 - protein, 9 aa, synthetic construct
GGNGTDLLR

SEQ ID NO: 47618 - protein, 9 aa, synthetic construct
GGNGTDELA

SEQ ID NO: 47619 - protein, 9 aa, synthetic construct
GGNGSDWID

SEQ ID NO: 47620 - protein, 9 aa, synthetic construct
GGNGSDWMV

SEQ ID NO: 47621 - protein, 9 aa, synthetic construct
GGNGSDYFD

SEQ ID NO: 47622 - protein, 9 aa, synthetic construct
GGNGSDYFI

SEQ ID NO: 47623 - protein, 9 aa, synthetic construct
GGNGSDYLD

SEQ ID NO: 47624 - protein, 9 aa, synthetic construct
GGNGSDYLE

SEQ ID NO: 47625 - protein, 9 aa, synthetic construct
GGNGSDYLS

SEQ ID NO: 47626 - protein, 9 aa, synthetic construct
GGNGSDYVD

SEQ ID NO: 47627 - protein, 9 aa, synthetic construct
GGNGSDYVK

SEQ ID NO: 47628 - protein, 9 aa, synthetic construct
GGNGTDALK

SEQ ID NO: 47629 - protein, 9 aa, synthetic construct
GGNGTDALY

SEQ ID NO: 47630 - protein, 9 aa, synthetic construct
GGNGTDDLN

SEQ ID NO: 47631 - protein, 9 aa, synthetic construct
GGNGTDDLR

SEQ ID NO: 47632 - protein, 9 aa, synthetic construct
GGNGTDELY

SEQ ID NO: 47633 - protein, 9 aa, synthetic construct
GGNGTDLLL

SEQ ID NO: 47634 - protein, 9 aa, synthetic construct
GGNGTDFID

SEQ ID NO: 47635 - protein, 9 aa, synthetic construct
GGNGTDFLV

SEQ ID NO: 47636 - protein, 9 aa, synthetic construct
GGNGTDGLF

SEQ ID NO: 47637 - protein, 9 aa, synthetic construct
GGNGTDHAD

SEQ ID NO: 47638 - protein, 9 aa, synthetic construct
GGNGTDHLF

SEQ ID NO: 47639 - protein, 9 aa, synthetic construct
GGNGTDIAR

SEQ ID NO: 47640 - protein, 9 aa, synthetic construct
GGNGTDILD

SEQ ID NO: 47641 - protein, 9 aa, synthetic construct
GGNGTDILG

SEQ ID NO: 47642 - protein, 9 aa, synthetic construct
GGNGTDILS

SEQ ID NO: 47643 - protein, 9 aa, synthetic construct
GGNGTDIMS

SEQ ID NO: 47644 - protein, 9 aa, synthetic construct
GGNGTDIYD

SEQ ID NO: 47645 - protein, 9 aa, synthetic construct
GGNGTDKAY

SEQ ID NO: 47646 - protein, 9 aa, synthetic construct
GGNGTDKLD

SEQ ID NO: 47647 - protein, 9 aa, synthetic construct
GGNGTDYLF

SEQ ID NO: 47648 - protein, 9 aa, synthetic construct
GGNGTDYLY

SEQ ID NO: 47649 - protein, 9 aa, synthetic construct
GGNGYDAAM

SEQ ID NO: 47650 - protein, 9 aa, synthetic construct
GGNGVDALD

SEQ ID NO: 47651 - protein, 9 aa, synthetic construct
GGNGVDTLR

SEQ ID NO: 47652 - protein, 9 aa, synthetic construct
GGNGVDTVT

SEQ ID NO: 47653 - protein, 9 aa, synthetic construct
GGNGVDTYV

SEQ ID NO: 47654 - protein, 9 aa, synthetic construct
GGNGVDVAA

SEQ ID NO: 47655 - protein, 9 aa, synthetic construct
GGNGVDVLD

SEQ ID NO: 47656 - protein, 9 aa, synthetic construct
GGNGVDVLQ

SEQ ID NO: 47657 - protein, 9 aa, synthetic construct
GGNGVDVLT

SEQ ID NO: 47658 - protein, 9 aa, synthetic construct
GGNGVDWAL

SEQ ID NO: 47659 - protein, 9 aa, synthetic construct
GGNGVDWLF

SEQ ID NO: 47660 - protein, 9 aa, synthetic construct
GGNGVDYIM

SEQ ID NO: 47661 - protein, 9 aa, synthetic construct
GGNGVDYLW

SEQ ID NO: 47662 - protein, 9 aa, synthetic construct
GGNGVDYVT

SEQ ID NO: 47663 - protein, 9 aa, synthetic construct
GGNGWDELF

SEQ ID NO: 47664 - protein, 9 aa, synthetic construct
GGNGWDFLD

SEQ ID NO: 47665 - protein, 9 aa, synthetic construct
GGNGWDHLT

SEQ ID NO: 47666 - protein, 9 aa, synthetic construct
GGNGWDILR

SEQ ID NO: 47667 - protein, 9 aa, synthetic construct
GGNGWDKIF

SEQ ID NO: 47668 - protein, 9 aa, synthetic construct
GGNGWDKLT

SEQ ID NO: 47669 - protein, 9 aa, synthetic construct
GGNGWDLLT

SEQ ID NO: 47670 - protein, 9 aa, synthetic construct
GGNGWDNMH

SEQ ID NO: 47671 - protein, 9 aa, synthetic construct
GGNGWDQLH

SEQ ID NO: 47672 - protein, 9 aa, synthetic construct
GGNGWDQMT

SEQ ID NO: 47673 - protein, 9 aa, synthetic construct
GGNGWDSLY

SEQ ID NO: 47674 - protein, 9 aa, synthetic construct
GGNGWDTAS

SEQ ID NO: 47675 - protein, 9 aa, synthetic construct
GGNGWDTLD

SEQ ID NO: 47676 - protein, 9 aa, synthetic construct
GGNGWDTLI

SEQ ID NO: 47677 - protein, 9 aa, synthetic construct
GGNGWDTVF

SEQ ID NO: 47678 - protein, 9 aa, synthetic construct
GGNGWDVLE

SEQ ID NO: 47679 - protein, 9 aa, synthetic construct
GGNGWDVLQ

SEQ ID NO: 47680 - protein, 9 aa, synthetic construct
GGNGVDTLN

SEQ ID NO: 47681 - protein, 9 aa, synthetic construct
GGNGVDTLA

SEQ ID NO: 47682 - protein, 9 aa, synthetic construct
GGNGVDTIN

SEQ ID NO: 47683 - protein, 9 aa, synthetic construct
GGNGVDNLA

SEQ ID NO: 47684 - protein, 9 aa, synthetic construct
GGNGVDALN

SEQ ID NO: 47685 - protein, 9 aa, synthetic construct
GGNGVDELQ

SEQ ID NO: 47686 - protein, 9 aa, synthetic construct
GGNGVDELR

SEQ ID NO: 47687 - protein, 9 aa, synthetic construct
GGNGVDGLR

SEQ ID NO: 47688 - protein, 9 aa, synthetic construct
GGNGVDIAI

SEQ ID NO: 47689 - protein, 9 aa, synthetic construct
GGNGVDIAS

SEQ ID NO: 47690 - protein, 9 aa, synthetic construct
GGNGVDILI

SEQ ID NO: 47691 - protein, 9 aa, synthetic construct
GGNGVDIMV

SEQ ID NO: 47692 - protein, 9 aa, synthetic construct
GGNGVDLIF

SEQ ID NO: 47693 - protein, 9 aa, synthetic construct
GGNGVDLIQ

SEQ ID NO: 47694 - protein, 9 aa, synthetic construct
GGNGVDLLH

SEQ ID NO: 47695 - protein, 9 aa, synthetic construct
GGNGVDLLS

SEQ ID NO: 47696 - protein, 9 aa, synthetic construct
GGNGVDLLY

SEQ ID NO: 47697 - protein, 9 aa, synthetic construct
GGNGVDNLQ

SEQ ID NO: 47698 - protein, 9 aa, synthetic construct
GGNGVDTFR

SEQ ID NO: 47699 - protein, 9 aa, synthetic construct
GGNGVDNVI

SEQ ID NO: 47700 - protein, 9 aa, synthetic construct
GGNGVDNVM

SEQ ID NO: 47701 - protein, 9 aa, synthetic construct
GGNGVDQIW

SEQ ID NO: 47702 - protein, 9 aa, synthetic construct
GGNGVDRLD

SEQ ID NO: 47703 - protein, 9 aa, synthetic construct
GGNGVDRLF

SEQ ID NO: 47704 - protein, 9 aa, synthetic construct
GGNGVDRLR

SEQ ID NO: 47705 - protein, 9 aa, synthetic construct
GGNGVDRLV

SEQ ID NO: 47706 - protein, 9 aa, synthetic construct
GGNGVDRMA

SEQ ID NO: 47707 - protein, 9 aa, synthetic construct
GGNGVDRVI

SEQ ID NO: 47708 - protein, 9 aa, synthetic construct
GGNGVDSLT

SEQ ID NO: 47709 - protein, 9 aa, synthetic construct
GGNGVDSLY

SEQ ID NO: 47710 - protein, 9 aa, synthetic construct
GGNGVDTAN

SEQ ID NO: 47711 - protein, 9 aa, synthetic construct
GGNGVDTAS

SEQ ID NO: 47712 - protein, 9 aa, synthetic construct
GGNGSDWAS

SEQ ID NO: 47713 - protein, 9 aa, synthetic construct
GGNGSDVVS

SEQ ID NO: 47714 - protein, 9 aa, synthetic construct
GGNGSDVLT

SEQ ID NO: 47715 - protein, 9 aa, synthetic construct
GGNGSDVLS

SEQ ID NO: 47716 - protein, 9 aa, synthetic construct
GGNGSDFLE

SEQ ID NO: 47717 - protein, 9 aa, synthetic construct
GGNGSDFLK

SEQ ID NO: 47718 - protein, 9 aa, synthetic construct
GGNGSDFYV

SEQ ID NO: 47719 - protein, 9 aa, synthetic construct
GGNGSDHLA

SEQ ID NO: 47720 - protein, 9 aa, synthetic construct
GGNGSDHLL

SEQ ID NO: 47721 - protein, 9 aa, synthetic construct
GGNGSDHLR

SEQ ID NO: 47722 - protein, 9 aa, synthetic construct
GGNGSDHVS

SEQ ID NO: 47723 - protein, 9 aa, synthetic construct
GGNGSDHYF

SEQ ID NO: 47724 - protein, 9 aa, synthetic construct
GGNGSDIFL

SEQ ID NO: 47725 - protein, 9 aa, synthetic construct
GGNGSDIIA

SEQ ID NO: 47726 - protein, 9 aa, synthetic construct
GGNGSDIIS

SEQ ID NO: 47727 - protein, 9 aa, synthetic construct
GGNGSDIMA

SEQ ID NO: 47728 - protein, 9 aa, synthetic construct
GGNGSDIVA

SEQ ID NO: 47729 - protein, 9 aa, synthetic construct
GGNGSDIYM

SEQ ID NO: 47730 - protein, 9 aa, synthetic construct
GGNGSDKLL

SEQ ID NO: 47731 - protein, 9 aa, synthetic construct
GGNGSDKVF

SEQ ID NO: 47732 - protein, 9 aa, synthetic construct
GGNGSDLAF

SEQ ID NO: 47733 - protein, 9 aa, synthetic construct
GGNGSDLAS

SEQ ID NO: 47734 - protein, 9 aa, synthetic construct
GGNGSDLLN

SEQ ID NO: 47735 - protein, 9 aa, synthetic construct
GGNGSDLLR

SEQ ID NO: 47736 - protein, 9 aa, synthetic construct
GGNGSDLLV

SEQ ID NO: 47737 - protein, 9 aa, synthetic construct
GGNGSDLYY

SEQ ID NO: 47738 - protein, 9 aa, synthetic construct
GGNGSDMIK

SEQ ID NO: 47739 - protein, 9 aa, synthetic construct
GGNGSDMLD

SEQ ID NO: 47740 - protein, 9 aa, synthetic construct
GGNGSDMLF

SEQ ID NO: 47741 - protein, 9 aa, synthetic construct
GGNGSDMLK

SEQ ID NO: 47742 - protein, 9 aa, synthetic construct
GGNGSDNLD

SEQ ID NO: 47743 - protein, 9 aa, synthetic construct
GGNGSDNLF

SEQ ID NO: 47744 - protein, 9 aa, synthetic construct
GGNGSDNLS

SEQ ID NO: 47745 - protein, 9 aa, synthetic construct
GGNGSDFLA

SEQ ID NO: 47746 - protein, 9 aa, synthetic construct
GGNGSDFIN

SEQ ID NO: 47747 - protein, 9 aa, synthetic construct
GGNGSDFIL

SEQ ID NO: 47748 - protein, 9 aa, synthetic construct
GGNGSDALI

SEQ ID NO: 47749 - protein, 9 aa, synthetic construct
GGNGRDVLY

SEQ ID NO: 47750 - protein, 9 aa, synthetic construct
GGNGRDVMF

SEQ ID NO: 47751 - protein, 9 aa, synthetic construct
GGNGRDVMH

SEQ ID NO: 47752 - protein, 9 aa, synthetic construct
GGNGRDVML

SEQ ID NO: 47753 - protein, 9 aa, synthetic construct
GGNGRDVVD

SEQ ID NO: 47754 - protein, 9 aa, synthetic construct
GGNGRDWLE

SEQ ID NO: 47755 - protein, 9 aa, synthetic construct
GGNGRDWLQ

SEQ ID NO: 47756 - protein, 9 aa, synthetic construct
GGNGRDWLV

SEQ ID NO: 47757 - protein, 9 aa, synthetic construct
GGNGRDWLY

SEQ ID NO: 47758 - protein, 9 aa, synthetic construct
GGNGRDYLD

SEQ ID NO: 47759 - protein, 9 aa, synthetic construct
GGNGRDYLV

SEQ ID NO: 47760 - protein, 9 aa, synthetic construct
GGNGSDAFS

SEQ ID NO: 47761 - protein, 9 aa, synthetic construct
GGNGSDAIF

SEQ ID NO: 47762 - protein, 9 aa, synthetic construct
GGNGSDAMA

SEQ ID NO: 47763 - protein, 9 aa, synthetic construct
GGNGSDFII

SEQ ID NO: 47764 - protein, 9 aa, synthetic construct
GGNGSDAME

SEQ ID NO: 47765 - protein, 9 aa, synthetic construct
GGNGSDAYD

SEQ ID NO: 47766 - protein, 9 aa, synthetic construct
GGNGSDDIR

SEQ ID NO: 47767 - protein, 9 aa, synthetic construct
GGNGSDDLD

SEQ ID NO: 47768 - protein, 9 aa, synthetic construct
GGNGSDDLK

SEQ ID NO: 47769 - protein, 9 aa, synthetic construct
GGNGSDDYY

SEQ ID NO: 47770 - protein, 9 aa, synthetic construct
GGNGSDEFH

SEQ ID NO: 47771 - protein, 9 aa, synthetic construct
GGNGSDEFI

SEQ ID NO: 47772 - protein, 9 aa, synthetic construct
GGNGSDEIF

SEQ ID NO: 47773 - protein, 9 aa, synthetic construct
GGNGSDELN

SEQ ID NO: 47774 - protein, 9 aa, synthetic construct
GGNGSDELQ

SEQ ID NO: 47775 - protein, 9 aa, synthetic construct
GGNGSDELR

SEQ ID NO: 47776 - protein, 9 aa, synthetic construct
GGNGSDFAN

SEQ ID NO: 47777 - protein, 9 aa, synthetic construct
GGNGSDNVA

SEQ ID NO: 47778 - protein, 9 aa, synthetic construct
GGNGSDNVE

SEQ ID NO: 47779 - protein, 9 aa, synthetic construct
GGNGSDQFR

SEQ ID NO: 47780 - protein, 9 aa, synthetic construct
GGNGSDTYI

SEQ ID NO: 47781 - protein, 9 aa, synthetic construct
GGNGSDTIF

SEQ ID NO: 47782 - protein, 9 aa, synthetic construct
GGNGSDTIM

SEQ ID NO: 47783 - protein, 9 aa, synthetic construct
GGNGSDTIN

SEQ ID NO: 47784 - protein, 9 aa, synthetic construct
GGNGSDTIV

SEQ ID NO: 47785 - protein, 9 aa, synthetic construct
GGNGSDTLG

SEQ ID NO: 47786 - protein, 9 aa, synthetic construct
GGNGSDTLH

SEQ ID NO: 47787 - protein, 9 aa, synthetic construct
GGNGSDTLK

SEQ ID NO: 47788 - protein, 9 aa, synthetic construct
GGNGSDTMD

SEQ ID NO: 47789 - protein, 9 aa, synthetic construct
GGNGSDTVD

SEQ ID NO: 47790 - protein, 9 aa, synthetic construct
GGNGSDTVL

SEQ ID NO: 47791 - protein, 9 aa, synthetic construct
GGNGSDTVN

SEQ ID NO: 47792 - protein, 9 aa, synthetic construct
GGNGSDTVT

SEQ ID NO: 47793 - protein, 9 aa, synthetic construct
GGNGSDTYE

SEQ ID NO: 47794 - protein, 9 aa, synthetic construct
GGNGSDTYM

SEQ ID NO: 47795 - protein, 9 aa, synthetic construct
GGNGSDTAD

SEQ ID NO: 47796 - protein, 9 aa, synthetic construct
GGNGSDTYQ

SEQ ID NO: 47797 - protein, 9 aa, synthetic construct
GGNGSDVFA

SEQ ID NO: 47798 - protein, 9 aa, synthetic construct
GGNGSDVFE

SEQ ID NO: 47799 - protein, 9 aa, synthetic construct
GGNGSDVFF

SEQ ID NO: 47800 - protein, 9 aa, synthetic construct
GGNGSDVFH

SEQ ID NO: 47801 - protein, 9 aa, synthetic construct
GGNGSDVFL

SEQ ID NO: 47802 - protein, 9 aa, synthetic construct
GGNGSDVIA

SEQ ID NO: 47803 - protein, 9 aa, synthetic construct
GGNGSDVIF

SEQ ID NO: 47804 - protein, 9 aa, synthetic construct
GGNGSDVIN

SEQ ID NO: 47805 - protein, 9 aa, synthetic construct
GGNGSDVIS

SEQ ID NO: 47806 - protein, 9 aa, synthetic construct
GGNGSDVLA

SEQ ID NO: 47807 - protein, 9 aa, synthetic construct
GGNGSDVLI

SEQ ID NO: 47808 - protein, 9 aa, synthetic construct
GGNGSDVLL

SEQ ID NO: 47809 - protein, 9 aa, synthetic construct
GGNGSDTIE

SEQ ID NO: 47810 - protein, 9 aa, synthetic construct
GGNGSDSVS

SEQ ID NO: 47811 - protein, 9 aa, synthetic construct
GGNGSDQFY

SEQ ID NO: 47812 - protein, 9 aa, synthetic construct
GGNGSDRLS

SEQ ID NO: 47813 - protein, 9 aa, synthetic construct
GGNGSDQIK

SEQ ID NO: 47814 - protein, 9 aa, synthetic construct
GGNGSDQLD

SEQ ID NO: 47815 - protein, 9 aa, synthetic construct
GGNGSDQLI

SEQ ID NO: 47816 - protein, 9 aa, synthetic construct
GGNGSDQLW

SEQ ID NO: 47817 - protein, 9 aa, synthetic construct
GGNGSDQLY

SEQ ID NO: 47818 - protein, 9 aa, synthetic construct
GGNGSDQMF

SEQ ID NO: 47819 - protein, 9 aa, synthetic construct
GGNGSDRAS

SEQ ID NO: 47820 - protein, 9 aa, synthetic construct
GGNGSDRAT

SEQ ID NO: 47821 - protein, 9 aa, synthetic construct
GGNGSDRID

SEQ ID NO: 47822 - protein, 9 aa, synthetic construct
GGNGSDRIS

SEQ ID NO: 47823 - protein, 9 aa, synthetic construct
GGNGSDRIV

SEQ ID NO: 47824 - protein, 9 aa, synthetic construct
GGNGSDRLD

SEQ ID NO: 47825 - protein, 9 aa, synthetic construct
GGNGSDRLK

SEQ ID NO: 47826 - protein, 9 aa, synthetic construct
GGNGSDRMD

SEQ ID NO: 47827 - protein, 9 aa, synthetic construct
GGNGSDSVF

SEQ ID NO: 47828 - protein, 9 aa, synthetic construct
GGNGSDRMH

SEQ ID NO: 47829 - protein, 9 aa, synthetic construct
GGNGSDRMN

SEQ ID NO: 47830 - protein, 9 aa, synthetic construct
GGNGSDRVF

SEQ ID NO: 47831 - protein, 9 aa, synthetic construct
GGNGSDRYW

SEQ ID NO: 47832 - protein, 9 aa, synthetic construct
GGNGSDSAS

SEQ ID NO: 47833 - protein, 9 aa, synthetic construct
GGNGSDSAY

SEQ ID NO: 47834 - protein, 9 aa, synthetic construct
GGNGSDSIL

SEQ ID NO: 47835 - protein, 9 aa, synthetic construct
GGNGSDSLI

SEQ ID NO: 47836 - protein, 9 aa, synthetic construct
GGNGSDSLQ

SEQ ID NO: 47837 - protein, 9 aa, synthetic construct
GGNGSDSLV

SEQ ID NO: 47838 - protein, 9 aa, synthetic construct
GGNGSDSMS

SEQ ID NO: 47839 - protein, 9 aa, synthetic construct
GGNGSDSVA

SEQ ID NO: 47840 - protein, 9 aa, synthetic construct
GGNGSDSVD

SEQ ID NO: 47841 - protein, 9 aa, synthetic construct
GGNGWDYLD

SEQ ID NO: 47842 - protein, 9 aa, synthetic construct
GGNGYDALA

SEQ ID NO: 47843 - protein, 9 aa, synthetic construct
GGNGHDRFV

SEQ ID NO: 47844 - protein, 9 aa, synthetic construct
GGPGDDIML

SEQ ID NO: 47845 - protein, 9 aa, synthetic construct
GGPGDDEVR

SEQ ID NO: 47846 - protein, 9 aa, synthetic construct
GGPGDDFIA

SEQ ID NO: 47847 - protein, 9 aa, synthetic construct
GGPGDDFID

SEQ ID NO: 47848 - protein, 9 aa, synthetic construct
GGPGDDFIG

SEQ ID NO: 47849 - protein, 9 aa, synthetic construct
GGPGDDFIN

SEQ ID NO: 47850 - protein, 9 aa, synthetic construct
GGPGDDFIQ

SEQ ID NO: 47851 - protein, 9 aa, synthetic construct
GGPGDDFLA

SEQ ID NO: 47852 - protein, 9 aa, synthetic construct
GGPGDDFLD

SEQ ID NO: 47853 - protein, 9 aa, synthetic construct
GGPGDDFLE

SEQ ID NO: 47854 - protein, 9 aa, synthetic construct
GGPGDDFLG

SEQ ID NO: 47855 - protein, 9 aa, synthetic construct
GGPGDDFLI

SEQ ID NO: 47856 - protein, 9 aa, synthetic construct
GGPGDDFLW

SEQ ID NO: 47857 - protein, 9 aa, synthetic construct
GGPGDDFVA

SEQ ID NO: 47858 - protein, 9 aa, synthetic construct
GGPGDDFYV

SEQ ID NO: 47859 - protein, 9 aa, synthetic construct
GGPGDDGFY

SEQ ID NO: 47860 - protein, 9 aa, synthetic construct
GGPGDDGLF

SEQ ID NO: 47861 - protein, 9 aa, synthetic construct
GGPGDDGLI

SEQ ID NO: 47862 - protein, 9 aa, synthetic construct
GGPGDDGLL

SEQ ID NO: 47863 - protein, 9 aa, synthetic construct
GGPGDDGLR

SEQ ID NO: 47864 - protein, 9 aa, synthetic construct
GGPGDDHLH

SEQ ID NO: 47865 - protein, 9 aa, synthetic construct
GGPGDDHLR

SEQ ID NO: 47866 - protein, 9 aa, synthetic construct
GGPGDDHYT

SEQ ID NO: 47867 - protein, 9 aa, synthetic construct
GGPGDDIAH

SEQ ID NO: 47868 - protein, 9 aa, synthetic construct
GGPGDDIAS

SEQ ID NO: 47869 - protein, 9 aa, synthetic construct
GGPGDDIFI

SEQ ID NO: 47870 - protein, 9 aa, synthetic construct
GGPGDDIIN

SEQ ID NO: 47871 - protein, 9 aa, synthetic construct
GGPGDDILG

SEQ ID NO: 47872 - protein, 9 aa, synthetic construct
GGPGDDILL

SEQ ID NO: 47873 - protein, 9 aa, synthetic construct
GGPGDDILV

SEQ ID NO: 47874 - protein, 9 aa, synthetic construct
GGPGDDELN

SEQ ID NO: 47875 - protein, 9 aa, synthetic construct
GGPGDDELI

SEQ ID NO: 47876 - protein, 9 aa, synthetic construct
GGPGDDELH

SEQ ID NO: 47877 - protein, 9 aa, synthetic construct
GGPGDDAIW

SEQ ID NO: 47878 - protein, 9 aa, synthetic construct
GGPGADWIH

SEQ ID NO: 47879 - protein, 9 aa, synthetic construct
GGPGADWIQ

SEQ ID NO: 47880 - protein, 9 aa, synthetic construct
GGPGADWLE

SEQ ID NO: 47881 - protein, 9 aa, synthetic construct
GGPGADWLI

SEQ ID NO: 47882 - protein, 9 aa, synthetic construct
GGPGADWLW

SEQ ID NO: 47883 - protein, 9 aa, synthetic construct
GGPGADYFN

SEQ ID NO: 47884 - protein, 9 aa, synthetic construct
GGPGADYIL

SEQ ID NO: 47885 - protein, 9 aa, synthetic construct
GGPGADYLI

SEQ ID NO: 47886 - protein, 9 aa, synthetic construct
GGPGADYLN

SEQ ID NO: 47887 - protein, 9 aa, synthetic construct
GGPGADYML

SEQ ID NO: 47888 - protein, 9 aa, synthetic construct
GGPGCDKLF

SEQ ID NO: 47889 - protein, 9 aa, synthetic construct
GGPGDDAFD

SEQ ID NO: 47890 - protein, 9 aa, synthetic construct
GGPGDDAID

SEQ ID NO: 47891 - protein, 9 aa, synthetic construct
GGPGDDALA

SEQ ID NO: 47892 - protein, 9 aa, synthetic construct
GGPGDDELD

SEQ ID NO: 47893 - protein, 9 aa, synthetic construct
GGPGDDALE

SEQ ID NO: 47894 - protein, 9 aa, synthetic construct
GGPGDDALH

SEQ ID NO: 47895 - protein, 9 aa, synthetic construct
GGPGDDALI

SEQ ID NO: 47896 - protein, 9 aa, synthetic construct
GGPGDDALY

SEQ ID NO: 47897 - protein, 9 aa, synthetic construct
GGPGDDAMM

SEQ ID NO: 47898 - protein, 9 aa, synthetic construct
GGPGDDAYF

SEQ ID NO: 47899 - protein, 9 aa, synthetic construct
GGPGDDCLL

SEQ ID NO: 47900 - protein, 9 aa, synthetic construct
GGPGDDDID

SEQ ID NO: 47901 - protein, 9 aa, synthetic construct
GGPGDDDIM

SEQ ID NO: 47902 - protein, 9 aa, synthetic construct
GGPGDDDIY

SEQ ID NO: 47903 - protein, 9 aa, synthetic construct
GGPGDDDLF

SEQ ID NO: 47904 - protein, 9 aa, synthetic construct
GGPGDDDLQ

SEQ ID NO: 47905 - protein, 9 aa, synthetic construct
GGPGDDEAR

SEQ ID NO: 47906 - protein, 9 aa, synthetic construct
GGPGDDILW

SEQ ID NO: 47907 - protein, 9 aa, synthetic construct
GGPGDDIMS

SEQ ID NO: 47908 - protein, 9 aa, synthetic construct
GGNGYDELS

SEQ ID NO: 47909 - protein, 9 aa, synthetic construct
GGPGDDIVA

SEQ ID NO: 47910 - protein, 9 aa, synthetic construct
GGPGDDQIF

SEQ ID NO: 47911 - protein, 9 aa, synthetic construct
GGPGDDQIS

SEQ ID NO: 47912 - protein, 9 aa, synthetic construct
GGPGDDQIY

SEQ ID NO: 47913 - protein, 9 aa, synthetic construct
GGPGDDQLQ

SEQ ID NO: 47914 - protein, 9 aa, synthetic construct
GGPGDDQLS

SEQ ID NO: 47915 - protein, 9 aa, synthetic construct
GGPGDDQVF

SEQ ID NO: 47916 - protein, 9 aa, synthetic construct
GGPGDDRFV

SEQ ID NO: 47917 - protein, 9 aa, synthetic construct
GGPGDDRID

SEQ ID NO: 47918 - protein, 9 aa, synthetic construct
GGPGDDRIE

SEQ ID NO: 47919 - protein, 9 aa, synthetic construct
GGPGDDRIN

SEQ ID NO: 47920 - protein, 9 aa, synthetic construct
GGPGDDRIS

SEQ ID NO: 47921 - protein, 9 aa, synthetic construct
GGPGDDRIW

SEQ ID NO: 47922 - protein, 9 aa, synthetic construct
GGPGDDRLH

SEQ ID NO: 47923 - protein, 9 aa, synthetic construct
GGPGDDRLN

SEQ ID NO: 47924 - protein, 9 aa, synthetic construct
GGPGDDRMD

SEQ ID NO: 47925 - protein, 9 aa, synthetic construct
GGPGDDRMV

SEQ ID NO: 47926 - protein, 9 aa, synthetic construct
GGPGDDRVY

SEQ ID NO: 47927 - protein, 9 aa, synthetic construct
GGPGDDRYL

SEQ ID NO: 47928 - protein, 9 aa, synthetic construct
GGPGDDSAS

SEQ ID NO: 47929 - protein, 9 aa, synthetic construct
GGPGDDSIL

SEQ ID NO: 47930 - protein, 9 aa, synthetic construct
GGPGDDSIV

SEQ ID NO: 47931 - protein, 9 aa, synthetic construct
GGPGDDSLH

SEQ ID NO: 47932 - protein, 9 aa, synthetic construct
GGPGDDSVL

SEQ ID NO: 47933 - protein, 9 aa, synthetic construct
GGPGDDSYV

SEQ ID NO: 47934 - protein, 9 aa, synthetic construct
GGPGDDTAI

SEQ ID NO: 47935 - protein, 9 aa, synthetic construct
GGPGDDTAL

SEQ ID NO: 47936 - protein, 9 aa, synthetic construct
GGPGDDTFL

SEQ ID NO: 47937 - protein, 9 aa, synthetic construct
GGPGDDTFQ

SEQ ID NO: 47938 - protein, 9 aa, synthetic construct
GGPGDDTFV

SEQ ID NO: 47939 - protein, 9 aa, synthetic construct
GGPGDDPII

SEQ ID NO: 47940 - protein, 9 aa, synthetic construct
GGPGDDNLT

SEQ ID NO: 47941 - protein, 9 aa, synthetic construct
GGPGDDNIY

SEQ ID NO: 47942 - protein, 9 aa, synthetic construct
GGPGDDLLC

SEQ ID NO: 47943 - protein, 9 aa, synthetic construct
GGPGDDIYQ

SEQ ID NO: 47944 - protein, 9 aa, synthetic construct
GGPGDDKFT

SEQ ID NO: 47945 - protein, 9 aa, synthetic construct
GGPGDDKIY

SEQ ID NO: 47946 - protein, 9 aa, synthetic construct
GGPGDDKLD

SEQ ID NO: 47947 - protein, 9 aa, synthetic construct
GGPGDDKLF

SEQ ID NO: 47948 - protein, 9 aa, synthetic construct
GGPGDDKLN

SEQ ID NO: 47949 - protein, 9 aa, synthetic construct
GGPGDDLFL

SEQ ID NO: 47950 - protein, 9 aa, synthetic construct
GGPGDDLFM

SEQ ID NO: 47951 - protein, 9 aa, synthetic construct
GGPGDDLIA

SEQ ID NO: 47952 - protein, 9 aa, synthetic construct
GGPGDDLIR

SEQ ID NO: 47953 - protein, 9 aa, synthetic construct
GGPGDDLIS

SEQ ID NO: 47954 - protein, 9 aa, synthetic construct
GGPGDDLIV

SEQ ID NO: 47955 - protein, 9 aa, synthetic construct
GGPGDDLIW

SEQ ID NO: 47956 - protein, 9 aa, synthetic construct
GGPGDDLLR

SEQ ID NO: 47957 - protein, 9 aa, synthetic construct
GGPGDDNFN

SEQ ID NO: 47958 - protein, 9 aa, synthetic construct
GGPGDDLLT

SEQ ID NO: 47959 - protein, 9 aa, synthetic construct
GGPGDDLMF

SEQ ID NO: 47960 - protein, 9 aa, synthetic construct
GGPGDDLMY

SEQ ID NO: 47961 - protein, 9 aa, synthetic construct
GGPGDDLVH

SEQ ID NO: 47962 - protein, 9 aa, synthetic construct
GGPGDDLVK

SEQ ID NO: 47963 - protein, 9 aa, synthetic construct
GGPGDDMAK

SEQ ID NO: 47964 - protein, 9 aa, synthetic construct
GGPGDDMFM

SEQ ID NO: 47965 - protein, 9 aa, synthetic construct
GGPGDDMIS

SEQ ID NO: 47966 - protein, 9 aa, synthetic construct
GGPGDDMLD

SEQ ID NO: 47967 - protein, 9 aa, synthetic construct
GGPGDDMLG

SEQ ID NO: 47968 - protein, 9 aa, synthetic construct
GGPGDDMLS

SEQ ID NO: 47969 - protein, 9 aa, synthetic construct
GGPGDDMLV

SEQ ID NO: 47970 - protein, 9 aa, synthetic construct
GGPGDDMYI

SEQ ID NO: 47971 - protein, 9 aa, synthetic construct
GGPGADVVR

SEQ ID NO: 47972 - protein, 9 aa, synthetic construct
GGPGADVVI

SEQ ID NO: 47973 - protein, 9 aa, synthetic construct
GGPGADVMY

SEQ ID NO: 47974 - protein, 9 aa, synthetic construct
GGPGADVMS

SEQ ID NO: 47975 - protein, 9 aa, synthetic construct
GGPGADFLI

SEQ ID NO: 47976 - protein, 9 aa, synthetic construct
GGPGADFVR

SEQ ID NO: 47977 - protein, 9 aa, synthetic construct
GGPGADGME

SEQ ID NO: 47978 - protein, 9 aa, synthetic construct
GGPGADHLF

SEQ ID NO: 47979 - protein, 9 aa, synthetic construct
GGPGADHVV

SEQ ID NO: 47980 - protein, 9 aa, synthetic construct
GGPGADIFE

SEQ ID NO: 47981 - protein, 9 aa, synthetic construct
GGPGADIFI

SEQ ID NO: 47982 - protein, 9 aa, synthetic construct
GGPGADIIY

SEQ ID NO: 47983 - protein, 9 aa, synthetic construct
GGPGADILA

SEQ ID NO: 47984 - protein, 9 aa, synthetic construct
GGPGADILR

SEQ ID NO: 47985 - protein, 9 aa, synthetic construct
GGPGADILV

SEQ ID NO: 47986 - protein, 9 aa, synthetic construct
GGPGADIMT

SEQ ID NO: 47987 - protein, 9 aa, synthetic construct
GGPGADIYE

SEQ ID NO: 47988 - protein, 9 aa, synthetic construct
GGPGADIYV

SEQ ID NO: 47989 - protein, 9 aa, synthetic construct
GGPGADKMT

SEQ ID NO: 47990 - protein, 9 aa, synthetic construct
GGPGADLAI

SEQ ID NO: 47991 - protein, 9 aa, synthetic construct
GGPGADLFI

SEQ ID NO: 47992 - protein, 9 aa, synthetic construct
GGPGADLFR

SEQ ID NO: 47993 - protein, 9 aa, synthetic construct
GGPGADLIE

SEQ ID NO: 47994 - protein, 9 aa, synthetic construct
GGPGADLIR

SEQ ID NO: 47995 - protein, 9 aa, synthetic construct
GGPGADLLA

SEQ ID NO: 47996 - protein, 9 aa, synthetic construct
GGPGADLLG

SEQ ID NO: 47997 - protein, 9 aa, synthetic construct
GGPGADLLH

SEQ ID NO: 47998 - protein, 9 aa, synthetic construct
GGPGADLLL

SEQ ID NO: 47999 - protein, 9 aa, synthetic construct
GGPGADLLM

SEQ ID NO: 48000 - protein, 9 aa, synthetic construct
GGPGADLLN

SEQ ID NO: 48001 - protein, 9 aa, synthetic construct
GGPGADLLR

SEQ ID NO: 48002 - protein, 9 aa, synthetic construct
GGPGADLLV

SEQ ID NO: 48003 - protein, 9 aa, synthetic construct
GGPGADLMI

SEQ ID NO: 48004 - protein, 9 aa, synthetic construct
GGPGADFID

SEQ ID NO: 48005 - protein, 9 aa, synthetic construct
GGPGADEMR

SEQ ID NO: 48006 - protein, 9 aa, synthetic construct
GGPGADELV

SEQ ID NO: 48007 - protein, 9 aa, synthetic construct
GGNGYDTLA

SEQ ID NO: 48008 - protein, 9 aa, synthetic construct
GGNGYDFAS

SEQ ID NO: 48009 - protein, 9 aa, synthetic construct
GGNGYDFMN

SEQ ID NO: 48010 - protein, 9 aa, synthetic construct
GGNGYDIVS

SEQ ID NO: 48011 - protein, 9 aa, synthetic construct
GGNGYDLAS

SEQ ID NO: 48012 - protein, 9 aa, synthetic construct
GGNGYDLIT

SEQ ID NO: 48013 - protein, 9 aa, synthetic construct
GGNGYDLLD

SEQ ID NO: 48014 - protein, 9 aa, synthetic construct
GGNGYDLMI

SEQ ID NO: 48015 - protein, 9 aa, synthetic construct
GGNGYDRLF

SEQ ID NO: 48016 - protein, 9 aa, synthetic construct
GGNGYDRLT

SEQ ID NO: 48017 - protein, 9 aa, synthetic construct
GGNGYDRMW

SEQ ID NO: 48018 - protein, 9 aa, synthetic construct
GGNGYDSLT

SEQ ID NO: 48019 - protein, 9 aa, synthetic construct
GGNGYDSLW

SEQ ID NO: 48020 - protein, 9 aa, synthetic construct
GGNGYDTAS

SEQ ID NO: 48021 - protein, 9 aa, synthetic construct
GGNGYDTLF

SEQ ID NO: 48022 - protein, 9 aa, synthetic construct
GGPGADELA

SEQ ID NO: 48023 - protein, 9 aa, synthetic construct
GGNGYDTYA

SEQ ID NO: 48024 - protein, 9 aa, synthetic construct
GGNGYDTYI

SEQ ID NO: 48025 - protein, 9 aa, synthetic construct
GGNGYDVII

SEQ ID NO: 48026 - protein, 9 aa, synthetic construct
GGNGYDVLS

SEQ ID NO: 48027 - protein, 9 aa, synthetic construct
GGNGYDWLS

SEQ ID NO: 48028 - protein, 9 aa, synthetic construct
GGNGYDYLD

SEQ ID NO: 48029 - protein, 9 aa, synthetic construct
GGPGADAIY

SEQ ID NO: 48030 - protein, 9 aa, synthetic construct
GGPGADALD

SEQ ID NO: 48031 - protein, 9 aa, synthetic construct
GGPGADALE

SEQ ID NO: 48032 - protein, 9 aa, synthetic construct
GGPGADALQ

SEQ ID NO: 48033 - protein, 9 aa, synthetic construct
GGPGADALS

SEQ ID NO: 48034 - protein, 9 aa, synthetic construct
GGPGADAYV

SEQ ID NO: 48035 - protein, 9 aa, synthetic construct
GGPGADDID

SEQ ID NO: 48036 - protein, 9 aa, synthetic construct
GGPGADLMS

SEQ ID NO: 48037 - protein, 9 aa, synthetic construct
GGPGADLVG

SEQ ID NO: 48038 - protein, 9 aa, synthetic construct
GGPGADLVR

SEQ ID NO: 48039 - protein, 9 aa, synthetic construct
GGPGADTYG

SEQ ID NO: 48040 - protein, 9 aa, synthetic construct
GGPGADTFY

SEQ ID NO: 48041 - protein, 9 aa, synthetic construct
GGPGADTIE

SEQ ID NO: 48042 - protein, 9 aa, synthetic construct
GGPGADTIK

SEQ ID NO: 48043 - protein, 9 aa, synthetic construct
GGPGADTIY

SEQ ID NO: 48044 - protein, 9 aa, synthetic construct
GGPGADTLN

SEQ ID NO: 48045 - protein, 9 aa, synthetic construct
GGPGADTLW

SEQ ID NO: 48046 - protein, 9 aa, synthetic construct
GGPGADTLY

SEQ ID NO: 48047 - protein, 9 aa, synthetic construct
GGPGADTMA

SEQ ID NO: 48048 - protein, 9 aa, synthetic construct
GGPGADTMD

SEQ ID NO: 48049 - protein, 9 aa, synthetic construct
GGPGADTVD

SEQ ID NO: 48050 - protein, 9 aa, synthetic construct
GGPGADTVE

SEQ ID NO: 48051 - protein, 9 aa, synthetic construct
GGPGADTVI

SEQ ID NO: 48052 - protein, 9 aa, synthetic construct
GGPGADTVT

SEQ ID NO: 48053 - protein, 9 aa, synthetic construct
GGPGADVAF

SEQ ID NO: 48054 - protein, 9 aa, synthetic construct
GGPGADSMV

SEQ ID NO: 48055 - protein, 9 aa, synthetic construct
GGPGADVFK

SEQ ID NO: 48056 - protein, 9 aa, synthetic construct
GGPGADVIL

SEQ ID NO: 48057 - protein, 9 aa, synthetic construct
GGPGADVIT

SEQ ID NO: 48058 - protein, 9 aa, synthetic construct
GGPGADVLA

SEQ ID NO: 48059 - protein, 9 aa, synthetic construct
GGPGADVLF

SEQ ID NO: 48060 - protein, 9 aa, synthetic construct
GGPGADVLK

SEQ ID NO: 48061 - protein, 9 aa, synthetic construct
GGPGADVLL

SEQ ID NO: 48062 - protein, 9 aa, synthetic construct
GGPGADVLS

SEQ ID NO: 48063 - protein, 9 aa, synthetic construct
GGPGADVLY

SEQ ID NO: 48064 - protein, 9 aa, synthetic construct
GGPGADVMD

SEQ ID NO: 48065 - protein, 9 aa, synthetic construct
GGPGADVME

SEQ ID NO: 48066 - protein, 9 aa, synthetic construct
GGPGADVMK

SEQ ID NO: 48067 - protein, 9 aa, synthetic construct
GGPGADVMN

SEQ ID NO: 48068 - protein, 9 aa, synthetic construct
GGPGADTFT

SEQ ID NO: 48069 - protein, 9 aa, synthetic construct
GGPGADSMM

SEQ ID NO: 48070 - protein, 9 aa, synthetic construct
GGPGADMLE

SEQ ID NO: 48071 - protein, 9 aa, synthetic construct
GGPGADRFL

SEQ ID NO: 48072 - protein, 9 aa, synthetic construct
GGPGADMLM

SEQ ID NO: 48073 - protein, 9 aa, synthetic construct
GGPGADMLR

SEQ ID NO: 48074 - protein, 9 aa, synthetic construct
GGPGADNLD

SEQ ID NO: 48075 - protein, 9 aa, synthetic construct
GGPGADNLS

SEQ ID NO: 48076 - protein, 9 aa, synthetic construct
GGPGADNLT

SEQ ID NO: 48077 - protein, 9 aa, synthetic construct
GGPGADNMQ

SEQ ID NO: 48078 - protein, 9 aa, synthetic construct
GGPGADQFV

SEQ ID NO: 48079 - protein, 9 aa, synthetic construct
GGPGADQIT

SEQ ID NO: 48080 - protein, 9 aa, synthetic construct
GGPGADQLF

SEQ ID NO: 48081 - protein, 9 aa, synthetic construct
GGPGADQLH

SEQ ID NO: 48082 - protein, 9 aa, synthetic construct
GGPGADQLW

SEQ ID NO: 48083 - protein, 9 aa, synthetic construct
GGPGADQME

SEQ ID NO: 48084 - protein, 9 aa, synthetic construct
GGPGADRFD

SEQ ID NO: 48085 - protein, 9 aa, synthetic construct
GGPGADRFR

SEQ ID NO: 48086 - protein, 9 aa, synthetic construct
GGPGADSMF

SEQ ID NO: 48087 - protein, 9 aa, synthetic construct
GGPGADRID

SEQ ID NO: 48088 - protein, 9 aa, synthetic construct
GGPGADRIH

SEQ ID NO: 48089 - protein, 9 aa, synthetic construct
GGPGADRIN

SEQ ID NO: 48090 - protein, 9 aa, synthetic construct
GGPGADRLA

SEQ ID NO: 48091 - protein, 9 aa, synthetic construct
GGPGADRLL

SEQ ID NO: 48092 - protein, 9 aa, synthetic construct
GGPGADRMD

SEQ ID NO: 48093 - protein, 9 aa, synthetic construct
GGPGADRMI

SEQ ID NO: 48094 - protein, 9 aa, synthetic construct
GGPGADRMV

SEQ ID NO: 48095 - protein, 9 aa, synthetic construct
GGPGADRMY

SEQ ID NO: 48096 - protein, 9 aa, synthetic construct
GGPGADRVR

SEQ ID NO: 48097 - protein, 9 aa, synthetic construct
GGPGADSLE

SEQ ID NO: 48098 - protein, 9 aa, synthetic construct
GGPGADSLF

SEQ ID NO: 48099 - protein, 9 aa, synthetic construct
GGPGADSLR

SEQ ID NO: 48100 - protein, 9 aa, synthetic construct
GGNGRDVLV

SEQ ID NO: 48101 - protein, 9 aa, synthetic construct
GGNGRDVLI

SEQ ID NO: 48102 - protein, 9 aa, synthetic construct
GGNGRDVLH

SEQ ID NO: 48103 - protein, 9 aa, synthetic construct
GGNGNDELW

SEQ ID NO: 48104 - protein, 9 aa, synthetic construct
GGNGNDAIH

SEQ ID NO: 48105 - protein, 9 aa, synthetic construct
GGNGNDAIT

SEQ ID NO: 48106 - protein, 9 aa, synthetic construct
GGNGNDALA

SEQ ID NO: 48107 - protein, 9 aa, synthetic construct
GGNGNDALH

SEQ ID NO: 48108 - protein, 9 aa, synthetic construct
GGNGNDALV

SEQ ID NO: 48109 - protein, 9 aa, synthetic construct
GGNGNDAMF

SEQ ID NO: 48110 - protein, 9 aa, synthetic construct
GGNGNDAMS

SEQ ID NO: 48111 - protein, 9 aa, synthetic construct
GGNGNDAVA

SEQ ID NO: 48112 - protein, 9 aa, synthetic construct
GGNGNDAVI

SEQ ID NO: 48113 - protein, 9 aa, synthetic construct
GGNGNDAYY

SEQ ID NO: 48114 - protein, 9 aa, synthetic construct
GGNGNDCFV

SEQ ID NO: 48115 - protein, 9 aa, synthetic construct
GGNGNDDFR

SEQ ID NO: 48116 - protein, 9 aa, synthetic construct
GGNGNDDIE

SEQ ID NO: 48117 - protein, 9 aa, synthetic construct
GGNGNDDIS

SEQ ID NO: 48118 - protein, 9 aa, synthetic construct
GGNGNDDLD

SEQ ID NO: 48119 - protein, 9 aa, synthetic construct
GGNGNDDLH

SEQ ID NO: 48120 - protein, 9 aa, synthetic construct
GGNGNDDLN

SEQ ID NO: 48121 - protein, 9 aa, synthetic construct
GGNGNDDLQ

SEQ ID NO: 48122 - protein, 9 aa, synthetic construct
GGNGNDDMD

SEQ ID NO: 48123 - protein, 9 aa, synthetic construct
GGNGNDDMY

SEQ ID NO: 48124 - protein, 9 aa, synthetic construct
GGNGNDDVL

SEQ ID NO: 48125 - protein, 9 aa, synthetic construct
GGNGNDDVS

SEQ ID NO: 48126 - protein, 9 aa, synthetic construct
GGNGNDEIA

SEQ ID NO: 48127 - protein, 9 aa, synthetic construct
GGNGNDEIE

SEQ ID NO: 48128 - protein, 9 aa, synthetic construct
GGNGNDEIG

SEQ ID NO: 48129 - protein, 9 aa, synthetic construct
GGNGNDEIR

SEQ ID NO: 48130 - protein, 9 aa, synthetic construct
GGNGNDEIV

SEQ ID NO: 48131 - protein, 9 aa, synthetic construct
GGNGNDELA

SEQ ID NO: 48132 - protein, 9 aa, synthetic construct
GGNGNDELD

SEQ ID NO: 48133 - protein, 9 aa, synthetic construct
GGNGNDAID

SEQ ID NO: 48134 - protein, 9 aa, synthetic construct
GGNGNDAAY

SEQ ID NO: 48135 - protein, 9 aa, synthetic construct
GGNGMDVLT

SEQ ID NO: 48136 - protein, 9 aa, synthetic construct
GGNGLDVAQ

SEQ ID NO: 48137 - protein, 9 aa, synthetic construct
GGNGLDRLT

SEQ ID NO: 48138 - protein, 9 aa, synthetic construct
GGNGLDRYD

SEQ ID NO: 48139 - protein, 9 aa, synthetic construct
GGNGLDSLF

SEQ ID NO: 48140 - protein, 9 aa, synthetic construct
GGNGLDTAA

SEQ ID NO: 48141 - protein, 9 aa, synthetic construct
GGNGLDTFI

SEQ ID NO: 48142 - protein, 9 aa, synthetic construct
GGNGLDTFS

SEQ ID NO: 48143 - protein, 9 aa, synthetic construct
GGNGLDTIN

SEQ ID NO: 48144 - protein, 9 aa, synthetic construct
GGNGLDTIS

SEQ ID NO: 48145 - protein, 9 aa, synthetic construct
GGNGLDTLD

SEQ ID NO: 48146 - protein, 9 aa, synthetic construct
GGNGLDTLI

SEQ ID NO: 48147 - protein, 9 aa, synthetic construct
GGNGLDTLQ

SEQ ID NO: 48148 - protein, 9 aa, synthetic construct
GGNGLDTLY

SEQ ID NO: 48149 - protein, 9 aa, synthetic construct
GGNGLDTMR

SEQ ID NO: 48150 - protein, 9 aa, synthetic construct
GGNGLDVLL

SEQ ID NO: 48151 - protein, 9 aa, synthetic construct
GGNGMDVLS

SEQ ID NO: 48152 - protein, 9 aa, synthetic construct
GGNGLDYAT

SEQ ID NO: 48153 - protein, 9 aa, synthetic construct
GGNGMDFLI

SEQ ID NO: 48154 - protein, 9 aa, synthetic construct
GGNGMDLIA

SEQ ID NO: 48155 - protein, 9 aa, synthetic construct
GGNGMDLIN

SEQ ID NO: 48156 - protein, 9 aa, synthetic construct
GGNGMDLLF

SEQ ID NO: 48157 - protein, 9 aa, synthetic construct
GGNGMDSLE

SEQ ID NO: 48158 - protein, 9 aa, synthetic construct
GGNGMDTID

SEQ ID NO: 48159 - protein, 9 aa, synthetic construct
GGNGMDTIG

SEQ ID NO: 48160 - protein, 9 aa, synthetic construct
GGNGMDTIS

SEQ ID NO: 48161 - protein, 9 aa, synthetic construct
GGNGMDTLI

SEQ ID NO: 48162 - protein, 9 aa, synthetic construct
GGNGMDTLN

SEQ ID NO: 48163 - protein, 9 aa, synthetic construct
GGNGMDTMF

SEQ ID NO: 48164 - protein, 9 aa, synthetic construct
GGNGMDVLN

SEQ ID NO: 48165 - protein, 9 aa, synthetic construct
GGNGNDELV

SEQ ID NO: 48166 - protein, 9 aa, synthetic construct
GGNGNDEYY

SEQ ID NO: 48167 - protein, 9 aa, synthetic construct
GGNGRDVLC

SEQ ID NO: 48168 - protein, 9 aa, synthetic construct
GGNGNDFAR

SEQ ID NO: 48169 - protein, 9 aa, synthetic construct
GGNGNDIIT

SEQ ID NO: 48170 - protein, 9 aa, synthetic construct
GGNGNDILG

SEQ ID NO: 48171 - protein, 9 aa, synthetic construct
GGNGNDIMA

SEQ ID NO: 48172 - protein, 9 aa, synthetic construct
GGNGNDIML

SEQ ID NO: 48173 - protein, 9 aa, synthetic construct
GGNGNDIMY

SEQ ID NO: 48174 - protein, 9 aa, synthetic construct
GGNGNDIVD

SEQ ID NO: 48175 - protein, 9 aa, synthetic construct
GGNGNDIVE

SEQ ID NO: 48176 - protein, 9 aa, synthetic construct
GGNGNDIVF

SEQ ID NO: 48177 - protein, 9 aa, synthetic construct
GGNGNDIVK

SEQ ID NO: 48178 - protein, 9 aa, synthetic construct
GGNGNDIVL

SEQ ID NO: 48179 - protein, 9 aa, synthetic construct
GGNGNDIVN

SEQ ID NO: 48180 - protein, 9 aa, synthetic construct
GGNGNDIVV

SEQ ID NO: 48181 - protein, 9 aa, synthetic construct
GGNGNDIYL

SEQ ID NO: 48182 - protein, 9 aa, synthetic construct
GGNGNDKIE

SEQ ID NO: 48183 - protein, 9 aa, synthetic construct
GGNGNDKII

SEQ ID NO: 48184 - protein, 9 aa, synthetic construct
GGNGNDKIN

SEQ ID NO: 48185 - protein, 9 aa, synthetic construct
GGNGNDKLK

SEQ ID NO: 48186 - protein, 9 aa, synthetic construct
GGNGNDKLR

SEQ ID NO: 48187 - protein, 9 aa, synthetic construct
GGNGNDKMT

SEQ ID NO: 48188 - protein, 9 aa, synthetic construct
GGNGNDKVY

SEQ ID NO: 48189 - protein, 9 aa, synthetic construct
GGNGNDLAF

SEQ ID NO: 48190 - protein, 9 aa, synthetic construct
GGNGNDLFD

SEQ ID NO: 48191 - protein, 9 aa, synthetic construct
GGNGNDLFI

SEQ ID NO: 48192 - protein, 9 aa, synthetic construct
GGNGNDLFR

SEQ ID NO: 48193 - protein, 9 aa, synthetic construct
GGNGNDLFY

SEQ ID NO: 48194 - protein, 9 aa, synthetic construct
GGNGNDLII

SEQ ID NO: 48195 - protein, 9 aa, synthetic construct
GGNGNDLIY

SEQ ID NO: 48196 - protein, 9 aa, synthetic construct
GGNGNDLLG

SEQ ID NO: 48197 - protein, 9 aa, synthetic construct
GGNGNDLME

SEQ ID NO: 48198 - protein, 9 aa, synthetic construct
GGNGNDIIR

SEQ ID NO: 48199 - protein, 9 aa, synthetic construct
GGNGNDIIH

SEQ ID NO: 48200 - protein, 9 aa, synthetic construct
GGNGNDIIC

SEQ ID NO: 48201 - protein, 9 aa, synthetic construct
GGNGNDGVG

SEQ ID NO: 48202 - protein, 9 aa, synthetic construct
GGNGNDFIE

SEQ ID NO: 48203 - protein, 9 aa, synthetic construct
GGNGNDFII

SEQ ID NO: 48204 - protein, 9 aa, synthetic construct
GGNGNDFLC

SEQ ID NO: 48205 - protein, 9 aa, synthetic construct
GGNGNDFLE

SEQ ID NO: 48206 - protein, 9 aa, synthetic construct
GGNGNDFLF

SEQ ID NO: 48207 - protein, 9 aa, synthetic construct
GGNGNDFLK

SEQ ID NO: 48208 - protein, 9 aa, synthetic construct
GGNGNDFML

SEQ ID NO: 48209 - protein, 9 aa, synthetic construct
GGNGNDFVN

SEQ ID NO: 48210 - protein, 9 aa, synthetic construct
GGNGNDFYI

SEQ ID NO: 48211 - protein, 9 aa, synthetic construct
GGNGNDGAY

SEQ ID NO: 48212 - protein, 9 aa, synthetic construct
GGNGNDGIV

SEQ ID NO: 48213 - protein, 9 aa, synthetic construct
GGNGNDGIY

SEQ ID NO: 48214 - protein, 9 aa, synthetic construct
GGNGNDGLH

SEQ ID NO: 48215 - protein, 9 aa, synthetic construct
GGNGNDHAE

SEQ ID NO: 48216 - protein, 9 aa, synthetic construct
GGNGNDIFN

SEQ ID NO: 48217 - protein, 9 aa, synthetic construct
GGNGNDHFV

SEQ ID NO: 48218 - protein, 9 aa, synthetic construct
GGNGNDHIF

SEQ ID NO: 48219 - protein, 9 aa, synthetic construct
GGNGNDHIG

SEQ ID NO: 48220 - protein, 9 aa, synthetic construct
GGNGNDHIN

SEQ ID NO: 48221 - protein, 9 aa, synthetic construct
GGNGNDHIR

SEQ ID NO: 48222 - protein, 9 aa, synthetic construct
GGNGNDHIS

SEQ ID NO: 48223 - protein, 9 aa, synthetic construct
GGNGNDHLH

SEQ ID NO: 48224 - protein, 9 aa, synthetic construct
GGNGNDHLI

SEQ ID NO: 48225 - protein, 9 aa, synthetic construct
GGNGNDHLT

SEQ ID NO: 48226 - protein, 9 aa, synthetic construct
GGNGNDHYF

SEQ ID NO: 48227 - protein, 9 aa, synthetic construct
GGNGNDHYY

SEQ ID NO: 48228 - protein, 9 aa, synthetic construct
GGNGNDIAY

SEQ ID NO: 48229 - protein, 9 aa, synthetic construct
GGNGNDIFE

SEQ ID NO: 48230 - protein, 9 aa, synthetic construct
GGNGLDRAD

SEQ ID NO: 48231 - protein, 9 aa, synthetic construct
GGNGLDQLY

SEQ ID NO: 48232 - protein, 9 aa, synthetic construct
GGNGLDNVV

SEQ ID NO: 48233 - protein, 9 aa, synthetic construct
GGNGLDNLF

SEQ ID NO: 48234 - protein, 9 aa, synthetic construct
GGNGHDYIY

SEQ ID NO: 48235 - protein, 9 aa, synthetic construct
GGNGHDYMC

SEQ ID NO: 48236 - protein, 9 aa, synthetic construct
GGNGIDAFN

SEQ ID NO: 48237 - protein, 9 aa, synthetic construct
GGNGIDAMF

SEQ ID NO: 48238 - protein, 9 aa, synthetic construct
GGNGIDAVS

SEQ ID NO: 48239 - protein, 9 aa, synthetic construct
GGNGIDELH

SEQ ID NO: 48240 - protein, 9 aa, synthetic construct
GGNGIDELY

SEQ ID NO: 48241 - protein, 9 aa, synthetic construct
GGNGIDIAQ

SEQ ID NO: 48242 - protein, 9 aa, synthetic construct
GGNGIDIID

SEQ ID NO: 48243 - protein, 9 aa, synthetic construct
GGNGIDILK

SEQ ID NO: 48244 - protein, 9 aa, synthetic construct
GGNGIDILL

SEQ ID NO: 48245 - protein, 9 aa, synthetic construct
GGNGIDKAI

SEQ ID NO: 48246 - protein, 9 aa, synthetic construct
GGNGIDKFL

SEQ ID NO: 48247 - protein, 9 aa, synthetic construct
GGNGIDKLS

SEQ ID NO: 48248 - protein, 9 aa, synthetic construct
GGNGIDNAI

SEQ ID NO: 48249 - protein, 9 aa, synthetic construct
GGNGIDNLI

SEQ ID NO: 48250 - protein, 9 aa, synthetic construct
GGNGIDQID

SEQ ID NO: 48251 - protein, 9 aa, synthetic construct
GGNGIDQIV

SEQ ID NO: 48252 - protein, 9 aa, synthetic construct
GGNGIDQLF

SEQ ID NO: 48253 - protein, 9 aa, synthetic construct
GGNGIDQLT

SEQ ID NO: 48254 - protein, 9 aa, synthetic construct
GGNGIDRLN

SEQ ID NO: 48255 - protein, 9 aa, synthetic construct
GGNGIDRLT

SEQ ID NO: 48256 - protein, 9 aa, synthetic construct
GGNGIDSAQ

SEQ ID NO: 48257 - protein, 9 aa, synthetic construct
GGNGIDSID

SEQ ID NO: 48258 - protein, 9 aa, synthetic construct
GGNGIDSIG

SEQ ID NO: 48259 - protein, 9 aa, synthetic construct
GGNGIDSLD

SEQ ID NO: 48260 - protein, 9 aa, synthetic construct
GGNGIDSLL

SEQ ID NO: 48261 - protein, 9 aa, synthetic construct
GGNGIDTFV

SEQ ID NO: 48262 - protein, 9 aa, synthetic construct
GGNGIDTFY

SEQ ID NO: 48263 - protein, 9 aa, synthetic construct
GGNGHDYIG

SEQ ID NO: 48264 - protein, 9 aa, synthetic construct
GGNGHDWVE

SEQ ID NO: 48265 - protein, 9 aa, synthetic construct
GGNGHDWLS

SEQ ID NO: 48266 - protein, 9 aa, synthetic construct
GGNGHDTAG

SEQ ID NO: 48267 - protein, 9 aa, synthetic construct
GGNGHDRFW

SEQ ID NO: 48268 - protein, 9 aa, synthetic construct
GGNGHDRIM

SEQ ID NO: 48269 - protein, 9 aa, synthetic construct
GGNGHDRLD

SEQ ID NO: 48270 - protein, 9 aa, synthetic construct
GGNGHDRLE

SEQ ID NO: 48271 - protein, 9 aa, synthetic construct
GGNGHDRLW

SEQ ID NO: 48272 - protein, 9 aa, synthetic construct
GGNGHDRLY

SEQ ID NO: 48273 - protein, 9 aa, synthetic construct
GGNGHDRMF

SEQ ID NO: 48274 - protein, 9 aa, synthetic construct
GGNGHDSIS

SEQ ID NO: 48275 - protein, 9 aa, synthetic construct
GGNGHDSLD

SEQ ID NO: 48276 - protein, 9 aa, synthetic construct
GGNGHDSLF

SEQ ID NO: 48277 - protein, 9 aa, synthetic construct
GGNGHDSLK

SEQ ID NO: 48278 - protein, 9 aa, synthetic construct
GGNGHDSLL

SEQ ID NO: 48279 - protein, 9 aa, synthetic construct
GGNGHDSLN

SEQ ID NO: 48280 - protein, 9 aa, synthetic construct
GGNGHDTIK

SEQ ID NO: 48281 - protein, 9 aa, synthetic construct
GGNGHDWLH

SEQ ID NO: 48282 - protein, 9 aa, synthetic construct
GGNGHDTIL

SEQ ID NO: 48283 - protein, 9 aa, synthetic construct
GGNGHDTLS

SEQ ID NO: 48284 - protein, 9 aa, synthetic construct
GGNGHDTVR

SEQ ID NO: 48285 - protein, 9 aa, synthetic construct
GGNGHDTYV

SEQ ID NO: 48286 - protein, 9 aa, synthetic construct
GGNGHDVIN

SEQ ID NO: 48287 - protein, 9 aa, synthetic construct
GGNGHDVLE

SEQ ID NO: 48288 - protein, 9 aa, synthetic construct
GGNGHDVLM

SEQ ID NO: 48289 - protein, 9 aa, synthetic construct
GGNGHDVLQ

SEQ ID NO: 48290 - protein, 9 aa, synthetic construct
GGNGHDVLV

SEQ ID NO: 48291 - protein, 9 aa, synthetic construct
GGNGHDVMG

SEQ ID NO: 48292 - protein, 9 aa, synthetic construct
GGNGHDVVS

SEQ ID NO: 48293 - protein, 9 aa, synthetic construct
GGNGHDWIV

SEQ ID NO: 48294 - protein, 9 aa, synthetic construct
GGNGHDWLD

SEQ ID NO: 48295 - protein, 9 aa, synthetic construct
GGNGIDTIF

SEQ ID NO: 48296 - protein, 9 aa, synthetic construct
GGNGIDTIK

SEQ ID NO: 48297 - protein, 9 aa, synthetic construct
GGNGIDTIQ

SEQ ID NO: 48298 - protein, 9 aa, synthetic construct
GGNGKDVAI

SEQ ID NO: 48299 - protein, 9 aa, synthetic construct
GGNGKDSIY

SEQ ID NO: 48300 - protein, 9 aa, synthetic construct
GGNGKDSLF

SEQ ID NO: 48301 - protein, 9 aa, synthetic construct
GGNGKDSLI

SEQ ID NO: 48302 - protein, 9 aa, synthetic construct
GGNGKDSLW

SEQ ID NO: 48303 - protein, 9 aa, synthetic construct
GGNGKDTFK

SEQ ID NO: 48304 - protein, 9 aa, synthetic construct
GGNGKDTFR

SEQ ID NO: 48305 - protein, 9 aa, synthetic construct
GGNGKDTID

SEQ ID NO: 48306 - protein, 9 aa, synthetic construct
GGNGKDTII

SEQ ID NO: 48307 - protein, 9 aa, synthetic construct
GGNGKDTLA

SEQ ID NO: 48308 - protein, 9 aa, synthetic construct
GGNGKDTLF

SEQ ID NO: 48309 - protein, 9 aa, synthetic construct
GGNGKDTLH

SEQ ID NO: 48310 - protein, 9 aa, synthetic construct
GGNGKDTLM

SEQ ID NO: 48311 - protein, 9 aa, synthetic construct
GGNGKDTLR

SEQ ID NO: 48312 - protein, 9 aa, synthetic construct
GGNGKDVLF

SEQ ID NO: 48313 - protein, 9 aa, synthetic construct
GGNGKDRLI

SEQ ID NO: 48314 - protein, 9 aa, synthetic construct
GGNGKDVLS

SEQ ID NO: 48315 - protein, 9 aa, synthetic construct
GGNGKDVLT

SEQ ID NO: 48316 - protein, 9 aa, synthetic construct
GGNGKDVLY

SEQ ID NO: 48317 - protein, 9 aa, synthetic construct
GGNGKDVVR

SEQ ID NO: 48318 - protein, 9 aa, synthetic construct
GGNGKDVVY

SEQ ID NO: 48319 - protein, 9 aa, synthetic construct
GGNGKDYLS

SEQ ID NO: 48320 - protein, 9 aa, synthetic construct
GGNGLDELS

SEQ ID NO: 48321 - protein, 9 aa, synthetic construct
GGNGLDELV

SEQ ID NO: 48322 - protein, 9 aa, synthetic construct
GGNGLDFVF

SEQ ID NO: 48323 - protein, 9 aa, synthetic construct
GGNGLDILD

SEQ ID NO: 48324 - protein, 9 aa, synthetic construct
GGNGLDKIN

SEQ ID NO: 48325 - protein, 9 aa, synthetic construct
GGNGLDKVI

SEQ ID NO: 48326 - protein, 9 aa, synthetic construct
GGNGLDLLV

SEQ ID NO: 48327 - protein, 9 aa, synthetic construct
GGNGKDRYL

SEQ ID NO: 48328 - protein, 9 aa, synthetic construct
GGNGKDRLD

SEQ ID NO: 48329 - protein, 9 aa, synthetic construct
GGNGIDTIW

SEQ ID NO: 48330 - protein, 9 aa, synthetic construct
GGNGIDVLT

SEQ ID NO: 48331 - protein, 9 aa, synthetic construct
GGNGIDTLI

SEQ ID NO: 48332 - protein, 9 aa, synthetic construct
GGNGIDTLK

SEQ ID NO: 48333 - protein, 9 aa, synthetic construct
GGNGIDTLL

SEQ ID NO: 48334 - protein, 9 aa, synthetic construct
GGNGIDTLT

SEQ ID NO: 48335 - protein, 9 aa, synthetic construct
GGNGIDTLV

SEQ ID NO: 48336 - protein, 9 aa, synthetic construct
GGNGIDTLY

SEQ ID NO: 48337 - protein, 9 aa, synthetic construct
GGNGIDTMV

SEQ ID NO: 48338 - protein, 9 aa, synthetic construct
GGNGIDTVD

SEQ ID NO: 48339 - protein, 9 aa, synthetic construct
GGNGIDTVS

SEQ ID NO: 48340 - protein, 9 aa, synthetic construct
GGNGIDTYI

SEQ ID NO: 48341 - protein, 9 aa, synthetic construct
GGNGIDTYL

SEQ ID NO: 48342 - protein, 9 aa, synthetic construct
GGNGIDVLE

SEQ ID NO: 48343 - protein, 9 aa, synthetic construct
GGNGIDVLL

SEQ ID NO: 48344 - protein, 9 aa, synthetic construct
GGNGIDYAS

SEQ ID NO: 48345 - protein, 9 aa, synthetic construct
GGNGKDQLF

SEQ ID NO: 48346 - protein, 9 aa, synthetic construct
GGNGIDYLY

SEQ ID NO: 48347 - protein, 9 aa, synthetic construct
GGNGKDALF

SEQ ID NO: 48348 - protein, 9 aa, synthetic construct
GGNGKDDLH

SEQ ID NO: 48349 - protein, 9 aa, synthetic construct
GGNGKDEIH

SEQ ID NO: 48350 - protein, 9 aa, synthetic construct
GGNGKDELN

SEQ ID NO: 48351 - protein, 9 aa, synthetic construct
GGNGKDELY

SEQ ID NO: 48352 - protein, 9 aa, synthetic construct
GGNGKDHLH

SEQ ID NO: 48353 - protein, 9 aa, synthetic construct
GGNGKDIFQ

SEQ ID NO: 48354 - protein, 9 aa, synthetic construct
GGNGKDILR

SEQ ID NO: 48355 - protein, 9 aa, synthetic construct
GGNGKDKLD

SEQ ID NO: 48356 - protein, 9 aa, synthetic construct
GGNGKDKLY

SEQ ID NO: 48357 - protein, 9 aa, synthetic construct
GGNGKDLMA

SEQ ID NO: 48358 - protein, 9 aa, synthetic construct
GGNGKDNLN

SEQ ID NO: 48359 - protein, 9 aa, synthetic construct
GGNGNDLMH

SEQ ID NO: 48360 - protein, 9 aa, synthetic construct
GGNGNDLML

SEQ ID NO: 48361 - protein, 9 aa, synthetic construct
GGNGNDLMS

SEQ ID NO: 48362 - protein, 9 aa, synthetic construct
GGNGPDRLT

SEQ ID NO: 48363 - protein, 9 aa, synthetic construct
GGNGQDRLV

SEQ ID NO: 48364 - protein, 9 aa, synthetic construct
GGNGQDRLY

SEQ ID NO: 48365 - protein, 9 aa, synthetic construct
GGNGQDSFA

SEQ ID NO: 48366 - protein, 9 aa, synthetic construct
GGNGQDSVY

SEQ ID NO: 48367 - protein, 9 aa, synthetic construct
GGNGQDTFV

SEQ ID NO: 48368 - protein, 9 aa, synthetic construct
GGNGQDTLD

SEQ ID NO: 48369 - protein, 9 aa, synthetic construct
GGNGQDTLE

SEQ ID NO: 48370 - protein, 9 aa, synthetic construct
GGNGQDTLG

SEQ ID NO: 48371 - protein, 9 aa, synthetic construct
GGNGQDTLS

SEQ ID NO: 48372 - protein, 9 aa, synthetic construct
GGNGQDVFD

SEQ ID NO: 48373 - protein, 9 aa, synthetic construct
GGNGQDVFT

SEQ ID NO: 48374 - protein, 9 aa, synthetic construct
GGNGQDVID

SEQ ID NO: 48375 - protein, 9 aa, synthetic construct
GGNGQDVLI

SEQ ID NO: 48376 - protein, 9 aa, synthetic construct
GGNGQDVLV

SEQ ID NO: 48377 - protein, 9 aa, synthetic construct
GGNGQDWAF

SEQ ID NO: 48378 - protein, 9 aa, synthetic construct
GGNGQDWLD

SEQ ID NO: 48379 - protein, 9 aa, synthetic construct
GGNGQDYLD

SEQ ID NO: 48380 - protein, 9 aa, synthetic construct
GGNGRDAFV

SEQ ID NO: 48381 - protein, 9 aa, synthetic construct
GGNGRDAIF

SEQ ID NO: 48382 - protein, 9 aa, synthetic construct
GGNGRDDLF

SEQ ID NO: 48383 - protein, 9 aa, synthetic construct
GGNGRDEID

SEQ ID NO: 48384 - protein, 9 aa, synthetic construct
GGNGRDELI

SEQ ID NO: 48385 - protein, 9 aa, synthetic construct
GGNGRDELL

SEQ ID NO: 48386 - protein, 9 aa, synthetic construct
GGNGRDELS

SEQ ID NO: 48387 - protein, 9 aa, synthetic construct
GGNGRDELY

SEQ ID NO: 48388 - protein, 9 aa, synthetic construct
GGNGRDFLN

SEQ ID NO: 48389 - protein, 9 aa, synthetic construct
GGNGRDFLR

SEQ ID NO: 48390 - protein, 9 aa, synthetic construct
GGNGRDFLV

SEQ ID NO: 48391 - protein, 9 aa, synthetic construct
GGNGRDFVR

SEQ ID NO: 48392 - protein, 9 aa, synthetic construct
GGNGQDRLF

SEQ ID NO: 48393 - protein, 9 aa, synthetic construct
GGNGQDRLA

SEQ ID NO: 48394 - protein, 9 aa, synthetic construct
GGNGQDQLY

SEQ ID NO: 48395 - protein, 9 aa, synthetic construct
GGNGQDDVS

SEQ ID NO: 48396 - protein, 9 aa, synthetic construct
GGNGPDTIQ

SEQ ID NO: 48397 - protein, 9 aa, synthetic construct
GGNGPDTLD

SEQ ID NO: 48398 - protein, 9 aa, synthetic construct
GGNGPDTLS

SEQ ID NO: 48399 - protein, 9 aa, synthetic construct
GGNGPDTME

SEQ ID NO: 48400 - protein, 9 aa, synthetic construct
GGNGPDTYI

SEQ ID NO: 48401 - protein, 9 aa, synthetic construct
GGNGPDVFV

SEQ ID NO: 48402 - protein, 9 aa, synthetic construct
GGNGPDVIH

SEQ ID NO: 48403 - protein, 9 aa, synthetic construct
GGNGPDVIR

SEQ ID NO: 48404 - protein, 9 aa, synthetic construct
GGNGPDWVV

SEQ ID NO: 48405 - protein, 9 aa, synthetic construct
GGNGQDALD

SEQ ID NO: 48406 - protein, 9 aa, synthetic construct
GGNGQDALY

SEQ ID NO: 48407 - protein, 9 aa, synthetic construct
GGNGQDDLI

SEQ ID NO: 48408 - protein, 9 aa, synthetic construct
GGNGQDDLQ

SEQ ID NO: 48409 - protein, 9 aa, synthetic construct
GGNGQDELN

SEQ ID NO: 48410 - protein, 9 aa, synthetic construct
GGNGQDQLQ

SEQ ID NO: 48411 - protein, 9 aa, synthetic construct
GGNGQDFLE

SEQ ID NO: 48412 - protein, 9 aa, synthetic construct
GGNGQDGIG

SEQ ID NO: 48413 - protein, 9 aa, synthetic construct
GGNGQDHLH

SEQ ID NO: 48414 - protein, 9 aa, synthetic construct
GGNGQDIAA

SEQ ID NO: 48415 - protein, 9 aa, synthetic construct
GGNGQDIIR

SEQ ID NO: 48416 - protein, 9 aa, synthetic construct
GGNGQDILI

SEQ ID NO: 48417 - protein, 9 aa, synthetic construct
GGNGQDILQ

SEQ ID NO: 48418 - protein, 9 aa, synthetic construct
GGNGQDKLY

SEQ ID NO: 48419 - protein, 9 aa, synthetic construct
GGNGQDLII

SEQ ID NO: 48420 - protein, 9 aa, synthetic construct
GGNGQDLLN

SEQ ID NO: 48421 - protein, 9 aa, synthetic construct
GGNGQDLLS

SEQ ID NO: 48422 - protein, 9 aa, synthetic construct
GGNGQDLVS

SEQ ID NO: 48423 - protein, 9 aa, synthetic construct
GGNGQDLVY

SEQ ID NO: 48424 - protein, 9 aa, synthetic construct
GGNGRDFVS

SEQ ID NO: 48425 - protein, 9 aa, synthetic construct
GGNGRDIFI

SEQ ID NO: 48426 - protein, 9 aa, synthetic construct
GGNGRDIFR

SEQ ID NO: 48427 - protein, 9 aa, synthetic construct
GGNGRDTFL

SEQ ID NO: 48428 - protein, 9 aa, synthetic construct
GGNGRDRLV

SEQ ID NO: 48429 - protein, 9 aa, synthetic construct
GGNGRDRMQ

SEQ ID NO: 48430 - protein, 9 aa, synthetic construct
GGNGRDRVY

SEQ ID NO: 48431 - protein, 9 aa, synthetic construct
GGNGRDSLA

SEQ ID NO: 48432 - protein, 9 aa, synthetic construct
GGNGRDSLG

SEQ ID NO: 48433 - protein, 9 aa, synthetic construct
GGNGRDSLI

SEQ ID NO: 48434 - protein, 9 aa, synthetic construct
GGNGRDSLK

SEQ ID NO: 48435 - protein, 9 aa, synthetic construct
GGNGRDSLL

SEQ ID NO: 48436 - protein, 9 aa, synthetic construct
GGNGRDSLT

SEQ ID NO: 48437 - protein, 9 aa, synthetic construct
GGNGRDSLV

SEQ ID NO: 48438 - protein, 9 aa, synthetic construct
GGNGRDSVF

SEQ ID NO: 48439 - protein, 9 aa, synthetic construct
GGNGRDSYY

SEQ ID NO: 48440 - protein, 9 aa, synthetic construct
GGNGRDTFF

SEQ ID NO: 48441 - protein, 9 aa, synthetic construct
GGNGRDTIF

SEQ ID NO: 48442 - protein, 9 aa, synthetic construct
GGNGRDRLS

SEQ ID NO: 48443 - protein, 9 aa, synthetic construct
GGNGRDTIK

SEQ ID NO: 48444 - protein, 9 aa, synthetic construct
GGNGRDTLF

SEQ ID NO: 48445 - protein, 9 aa, synthetic construct
GGNGRDTLH

SEQ ID NO: 48446 - protein, 9 aa, synthetic construct
GGNGRDTLM

SEQ ID NO: 48447 - protein, 9 aa, synthetic construct
GGNGRDTLN

SEQ ID NO: 48448 - protein, 9 aa, synthetic construct
GGNGRDTMT

SEQ ID NO: 48449 - protein, 9 aa, synthetic construct
GGNGRDTVF

SEQ ID NO: 48450 - protein, 9 aa, synthetic construct
GGNGRDTVY

SEQ ID NO: 48451 - protein, 9 aa, synthetic construct
GGNGRDVFA

SEQ ID NO: 48452 - protein, 9 aa, synthetic construct
GGNGRDVFS

SEQ ID NO: 48453 - protein, 9 aa, synthetic construct
GGNGRDVID

SEQ ID NO: 48454 - protein, 9 aa, synthetic construct
GGNGRDVII

SEQ ID NO: 48455 - protein, 9 aa, synthetic construct
GGNGRDVLA

SEQ ID NO: 48456 - protein, 9 aa, synthetic construct
GGNGRDRLT

SEQ ID NO: 48457 - protein, 9 aa, synthetic construct
GGNGRDRLN

SEQ ID NO: 48458 - protein, 9 aa, synthetic construct
GGNGRDIIS

SEQ ID NO: 48459 - protein, 9 aa, synthetic construct
GGNGRDLLN

SEQ ID NO: 48460 - protein, 9 aa, synthetic construct
GGNGRDILE

SEQ ID NO: 48461 - protein, 9 aa, synthetic construct
GGNGRDILF

SEQ ID NO: 48462 - protein, 9 aa, synthetic construct
GGNGRDILN

SEQ ID NO: 48463 - protein, 9 aa, synthetic construct
GGNGRDIVH

SEQ ID NO: 48464 - protein, 9 aa, synthetic construct
GGNGRDKIN

SEQ ID NO: 48465 - protein, 9 aa, synthetic construct
GGNGRDKLF

SEQ ID NO: 48466 - protein, 9 aa, synthetic construct
GGNGRDKLI

SEQ ID NO: 48467 - protein, 9 aa, synthetic construct
GGNGRDKLN

SEQ ID NO: 48468 - protein, 9 aa, synthetic construct
GGNGRDKMY

SEQ ID NO: 48469 - protein, 9 aa, synthetic construct
GGNGRDLIL

SEQ ID NO: 48470 - protein, 9 aa, synthetic construct
GGNGRDLIV

SEQ ID NO: 48471 - protein, 9 aa, synthetic construct
GGNGRDLLA

SEQ ID NO: 48472 - protein, 9 aa, synthetic construct
GGNGRDLLE

SEQ ID NO: 48473 - protein, 9 aa, synthetic construct
GGNGRDLLQ

SEQ ID NO: 48474 - protein, 9 aa, synthetic construct
GGNGRDRLA

SEQ ID NO: 48475 - protein, 9 aa, synthetic construct
GGNGRDLLR

SEQ ID NO: 48476 - protein, 9 aa, synthetic construct
GGNGRDLLS

SEQ ID NO: 48477 - protein, 9 aa, synthetic construct
GGNGRDLMS

SEQ ID NO: 48478 - protein, 9 aa, synthetic construct
GGNGRDLMT

SEQ ID NO: 48479 - protein, 9 aa, synthetic construct
GGNGRDLVS

SEQ ID NO: 48480 - protein, 9 aa, synthetic construct
GGNGRDMIK

SEQ ID NO: 48481 - protein, 9 aa, synthetic construct
GGNGRDMMT

SEQ ID NO: 48482 - protein, 9 aa, synthetic construct
GGNGRDNLR

SEQ ID NO: 48483 - protein, 9 aa, synthetic construct
GGNGRDQIF

SEQ ID NO: 48484 - protein, 9 aa, synthetic construct
GGNGRDQVR

SEQ ID NO: 48485 - protein, 9 aa, synthetic construct
GGNGRDRAY

SEQ ID NO: 48486 - protein, 9 aa, synthetic construct
GGNGRDRIR

SEQ ID NO: 48487 - protein, 9 aa, synthetic construct
GGNGRDRIY

SEQ ID NO: 48488 - protein, 9 aa, synthetic construct
GGNGPDTFV

SEQ ID NO: 48489 - protein, 9 aa, synthetic construct
GGNGPDRLN

SEQ ID NO: 48490 - protein, 9 aa, synthetic construct
GGNGNDLVF

SEQ ID NO: 48491 - protein, 9 aa, synthetic construct
GGNGPDRLC

SEQ ID NO: 48492 - protein, 9 aa, synthetic construct
GGNGNDRLM

SEQ ID NO: 48493 - protein, 9 aa, synthetic construct
GGNGNDRLR

SEQ ID NO: 48494 - protein, 9 aa, synthetic construct
GGNGNDRMN

SEQ ID NO: 48495 - protein, 9 aa, synthetic construct
GGNGNDRMT

SEQ ID NO: 48496 - protein, 9 aa, synthetic construct
GGNGNDRVG

SEQ ID NO: 48497 - protein, 9 aa, synthetic construct
GGNGNDRVI

SEQ ID NO: 48498 - protein, 9 aa, synthetic construct
GGNGNDRVS

SEQ ID NO: 48499 - protein, 9 aa, synthetic construct
GGNGNDRVT

SEQ ID NO: 48500 - protein, 9 aa, synthetic construct
GGNGNDSAD

SEQ ID NO: 48501 - protein, 9 aa, synthetic construct
GGNGNDSAF

SEQ ID NO: 48502 - protein, 9 aa, synthetic construct
GGNGNDSFG

SEQ ID NO: 48503 - protein, 9 aa, synthetic construct
GGNGNDSFR

SEQ ID NO: 48504 - protein, 9 aa, synthetic construct
GGNGNDSIA

SEQ ID NO: 48505 - protein, 9 aa, synthetic construct
GGNGNDSIG

SEQ ID NO: 48506 - protein, 9 aa, synthetic construct
GGNGNDSIK

SEQ ID NO: 48507 - protein, 9 aa, synthetic construct
GGNGNDSLK

SEQ ID NO: 48508 - protein, 9 aa, synthetic construct
GGNGNDSMA

SEQ ID NO: 48509 - protein, 9 aa, synthetic construct
GGNGNDSMF

SEQ ID NO: 48510 - protein, 9 aa, synthetic construct
GGNGNDSMS

SEQ ID NO: 48511 - protein, 9 aa, synthetic construct
GGNGNDSMV

SEQ ID NO: 48512 - protein, 9 aa, synthetic construct
GGNGNDSVA

SEQ ID NO: 48513 - protein, 9 aa, synthetic construct
GGNGNDSVD

SEQ ID NO: 48514 - protein, 9 aa, synthetic construct
GGNGNDSVH

SEQ ID NO: 48515 - protein, 9 aa, synthetic construct
GGNGNDSVI

SEQ ID NO: 48516 - protein, 9 aa, synthetic construct
GGNGNDSVN

SEQ ID NO: 48517 - protein, 9 aa, synthetic construct
GGNGNDSVQ

SEQ ID NO: 48518 - protein, 9 aa, synthetic construct
GGNGNDSVR

SEQ ID NO: 48519 - protein, 9 aa, synthetic construct
GGNGNDTAF

SEQ ID NO: 48520 - protein, 9 aa, synthetic construct
GGNGNDTAL

SEQ ID NO: 48521 - protein, 9 aa, synthetic construct
GGNGNDRIK

SEQ ID NO: 48522 - protein, 9 aa, synthetic construct
GGNGNDRII

(The sequence listing continues in the following parts.)